European Patent Application EP 4 520 821 A1 - sequence listing, part 10

SEQ ID NO: 15187 - RNA, 9550 nt, Homo sapiens
  source 1..9550: mol_type = other RNA
gctgggattacaggcatgagccactgcacctggtcctggctacattttgtattttttatagagatgggagtctcccaatgttgcccaggctggtcctgagctcttgagctcaagcaatctgcctgcctcagcctcccaaagtgctgggattaaaggtgtgagccaccgcacccagctggaaatttgttagacccctttccgcacttgatgttagacaacagacctataagcaattttatatcttctggcttactttttgtttgttttgctttggtttttgtatttcatggttgggagcaaggcaaaagtgccccaaggttttcggtgtttaagatctccgaagttttaggcccagatcacatatctaatgaatcaaacagacaggacgcaaacccatgcctccgtgacccaaagccccttcatgtataaaatgatgagccagggtcaagctccaggatgcccctgaaagttctagccattcttatggcatagcactgtacactgggacatgacttaatttctccacaggcttctcaaatcctaaaacacgtctctgtccacgcctgaggctcggtatcacaaagccttgtgaaaacgcctctcctgagagaactttcagcccccagacagccgctcattcccttcaagggctgtggtcccaggtcccgggccctagctgtgcttcagtgacatgattcaggagaacctcctccaaagcagcagggcaaaccctgttattttctgggagctgttgtccttgagtcattacctcacactcttagaacttcttccagtttctagagatgaaaatgcgactcagacagtctttgtgactaaggatagaagagaatataagggtgaacacaggacaccttgtggactgaggacataagttcgtaaaagctccctgggctgatgattttaatacaaaagagccaccagacacggttctgagtttaaaagtagaagaaatctggtccagtgtaaatcaagcttattaacgtaaagaattagtgcagaaaaattaaatgagtggatgaagaaaaaagtttggaaggaaaaaataatcctcctcactaccttttaccaaatgagcgttggcaacatgggttggagttgcctttatgcacataatttgccatgcctacattctttcagggcctacaataatgttcctagccatgtatttgaattaaccaggcccagaggataaaactttcaaattaaacacattcctaaaggatttcaggctcattgtgtatgcaccaaggaaacataacatcctaaaaataatacgtacacagagagaagcacattttccatgaacattaaagtggaatatgaattatgacccagctcatgggaatagacatctgattacatgcaaaatggagcttttgtaaataacatcagtcttcgtgagctaccacaattattatcaaccatttaattttattccctagcaactcatccatcgttgttaaaactgtccacttttgttttttaccttctgatgcatgaggctccgaattttataaagttcaccgttaaagctatgtagattaccagcccaacagcgaacgagttcacgaaattattagattcaccaaagcatatgctgcattgtatatctgctattttgggatgtattttgctggtgaattgctagaagcagcaaaattacaacggtagccattctgttcactttttatacaaaggaatcatgaaaatgtgtttaaactttcggtatttgggtatttaagtgcaaagtgactctcaagaaaatcaagtatacttctttctgtctccctggcctgcaatctttgacactattttatgaaataccatccataattccagttggtctatgtcatatataatacgcctgcctcataagtagtaaaataagccactttgtgccttcaccaattctatttcacaacaaagtcaagagacatgtttattaatagaactaaacttttattgatagaagtttaaacaggaatagatgaaggatgctgccaaatgcatcctttgcctgttcctattttaaactcaaaaaccagacacaagaagtacctatggctaatcttttgttctgggagaagttgctaggtggcacctctgaacaatgcctttaacaccttatgggagacctgacctcataaaatacgttgtattttctttcccttgaaattccatttcagtcagaggtgaggattttcattggcttccagaaacctttgagttttaactgcatcaggagtaagcttagaaagcctcctggcttgaagaattttctgaagttagccaagaaaaataagctacgatcaaggaggaaaagctggagtttcagttttctggagattgtacttcctggtaacataaaaacaaaagttaaattcagaaaaattcaactatgaagttagcatcacataaaaaacaatggaaaatatttaactatgcgcatatgtttgtacacaaacagaaatagatataaacagaccttaattagcattgtagactttaattatctttgtacagtaattgggaatggttttgttctgatttattccataatgcttactgtgttctgttaacaactcatttttttccccttccagcccataatagaaggcttttactgcatactttattacatctgcttctcatttaatgaccattgttctggtctgtcagagcgagtggctatacaacttcccaaatctgcaagattaagcaaatattttgacaatgtctagtttcttttttcctttttttcaaaacataccagataaaaataaaaagatttttacttacccacacaacgttaggagagtttttaatctaacgacaataaagaactaagcggcagcaaaatgtacttcatgtggcaaaatacatcaagcaattttctgtcccatttcacttaaaaagtcctaagaatctggtctgaatcacacagctggggttaatgggagcactcctggactgcagggaggttgtgggcccctgggcaaaccacgtggagaccttcaagcttctagaatgagacagaggccttctgctcattttggagggccccggcaggtaagctgaatgataggtgtctgaatcactcactatgaaatgtcatttttaaaaatggtcatgctacatacaaaattgcaataccactgatggcataaggaccagggtcataactctccccaaagaaggtggatacaaatacacaaacagaagcatttctaagcaactgggcagagagatacagagaaaagaggatacagcgaaaaatctattaacccataggcattcattaattctacaaatgatctaatggtgggaagcagaaaatacacaaataaaccaacaaaagcatgacatggacataaatgctaagagggaatggtatgtggaagatgctgcagtcagtggaatgagggaaaggggttaagaacagatgagctttcaagagacagtctatgcctttcagagtagtttaggaaaaaagttaccgaaagataactaggaacagaaaacaaggtgacagaaaggaccgcattaaccccagaagcataagcctcttaaaactttctggtggggagcctctccttggaggcagcaaccagggaaaattcccgcaaggaggtcctacgggagcagccagaattctactagaaagacaggaaagacatgacagggatgggtctgtaggagagcatcggcaaagatagcaagaggatgcaatcctctttagaggaagtagaggtttgccttgttgctattagattgcttcacatctccattggtttgcgtttactatagggcggaaagcacaaagcaggatatgtatgtgcttcaggaagcttaagtgcaaggcaatggggttcatttgtgagctactggcaaaccatttgtatttggggtgggcgtcccgtgcagcacgcctctggaacagtcccttcactgttaacaccactgactgggcccttaattggagcaggtctgcgcgttttaataaacatctttgatgagttctctggactgttccattaaacactcattctaccaaaaatgcctggtaattctctctaaaaatgttttcatgttaccgcttccaggtctttctaaagttaggcagtacaaagaaacaaaaatccaaaagacttgactttaatttagaagtctcaaagagagtgttcaccctagagcagagatttctaaagttgtagtattggactcgcttgcctccacccccacccctgcccttctcccaaaacaagaaaacaaagcagcatcaaagcttgaggtacagaacagaataaaacatgttggtgcagatttgctggcctcggtgaaaacaacctgaatcagtaggtcttggggtatcttcacttttaacaaacactacaggggattttgatgcagtcagttcaggaattaaattttgaaacacacttttgtcaggcggcaacagggtagatagcttaagaatggggtaggaagctagactataggaattcaaatcctagctcctctacttcctagctgtgtgaccttaggaaataaacactctgtgcttcagtctccttatcttcaaaatgggataatgggagcaatgtgtaagaattgaaaaatatgtaaagtacttagtactgtgccagacatgtcgtaagtgcatgaaaaatgttagccactattaacagtggattcatcccaaagtgatttcagctaatgagccaaatttgggtagaggaagtacgctgaagcagattccaaccaaaccaatgaatgaatacagctaagcataaaatagaatccttattaggtatcctcccaccatcatttcagtacggtcagcaccagtctataagctgtacagacatcctatacaatatcaatctcctgtagcacaatatatcctaacaatcctcttgggcacagacgcagccacagggcaggagacaaagcaacagaaccagcaagcacgcactctgctgcctcacttcatgggaatcccattcaacaccagtctaggaagagatgaccttggaatgcagatccagttaattcaattcaatgagcatttattgaacccttgtgatgtatcagagattcacctagatgctgaggataatacaaagagcaacaagaaaatcaccctgtcctcaaggaggtcataatctagtgggaaaaagagatacaagtaattgtaaggcaaggtggcctgagatgaatgctataatagaagatggaagaaggccatgcgaacacagagtaagtagtaattaactctgatgggggcagtcaggaaaggctttcctgaagagcagacatagcatgccattgtgagagatcaataaggcaagcctatgaaattgtttaatgactttatcattcatggaaacaacccagaaaaagcctgagggaccatctctgtctctgcattaacatgggtgtgtttaagatttgattaaatgtttgttgtttctgtaacatcgcatttaaaaaaaaaccaagtatgaacattcgtctattattctgatcttcttcaaagagagaaagagtcctagaaatacttttcttttttccaaagcaaaccctctgcattaatagcaaaagaagaatggcaagttatcgaacgtattatgaactagttagccaaagcgcaagtctgggaaggcccacatttgttttatgtagcaatgagacaaaatatgagagtttttttcttcttatatatggttgcctctttctacttgactataatcattaataatttctttggaccagcagaggaaacaggtattgatcacaataaaacattgcatccacaaacacttgctatagcaggttatggtctccatggaaaccctccaatagaaccaatctgaattcaatttcagaagtaatgagaacagataattttacactcaatcaatcactgtcagctgccgttatcagccaatcagtcattatgtcagtcagtcacactctcaacaaacttcttctgtggcatggtcagatgagaatgttttgacatccagaagcaacacgagaaaattggctcatctttcctggcaagatgccaaagacacagcactgcattgtgtttgctaaggcaataaacagtccaatcaaaatacactgtggtagcggaagattctaggcagcaatttcaataattgttatgatactgatggcagagacgtactttcgacccaaaagtcatacagtttaatcctctcatttaaacatgaagaaacagagcaccagagaagttcaagtatctgcccaaagctgcacagctaactggtggaaagcccacgactaaaacatgagcattctccccttccagtgctcatccaggatgccttgctgctgctcttcactgccttcctttttgaggcaagagggtaaagggatatttgaagattaggttctaattctaaacagagagccccaagcctgtgggagactcacgggatatttgtgaggcttgtgctttggagccaactcaaacctcttgctgtttggggttagctcgtccttggccaagtacaacttctggtttctaaggaggaacaaaagattttgaaacactacagggcaaccaaatcactgttacaaaatgacattttcgataagtttagtgcaggactatcaagaacacatggactgaattccctaaaaatgcttgggagagggaggtaaaatttgaggggaaaaatctggcaaaatacagttgggctcttgtcaacctcaaatgttagaaatgttggcatttgggaattgtgaagaatctgaaaggtgtctggtttctttcttttttctttttactgcattattgctttgtccatttctcagagacagttctctgaggctgaggttcacattcttccttggtaaaacagatggttgggaggccgaggcaggcagatcacgaggtcatgagttcgaggcaggcagatcacgaggtcaggagttcgagaccagcctgaccaacatggtgaaacctgtctctactaagaaaatacaaaaattagctgggtgtggtggtgcacacctgtaatcccagctactcaggaagctgaggcaggcgaatcacttgaacctgggaggtggacgttacagtgagccaagattgcaccactgtactccagcctgggcgacagagtgagactctgtctcaaaaaaaaaaaaaaaaaaatagatggaccagcttgatagtttgcaaacttcaatgtgcatgggaacttaccaaatctgttaaaaatgcaaatccccagatcccacctccagacattttcattcagcaggtgaggctgggcccaggaatctgcctttttaacaaaggacccaggtaattctgatgcactttctttgccaatcagtgttagaaaacattggttaactaatgctatttggtaaagaatttgggccattttgttgatggtagttttccaattacattcctccccaaacattccaacttcgtaaattgtgtgtatcacccatattacaagaacataattctaatggctatgatcacaagctttgatatatatatatatatatatatatatatatatatatatatatatatatataaaatatatgaaatatacattatagtgccactttctattagctgtaagtaggctttatcttaaataggtaggtggtatatgggacactaatacatcccatcagaatttgtctaaggcaaatgaggtgaaaaagcaaagcaagaatatgggttcaggcttgagctaaaactagtaattgcaaaaagaacagtttggaagctttcacatgaaatgcttgcttcatttctctagtctgcttgcctgacctcagctcacgatacctattttatcttctcgcaaaacattgatataaagctttttgcctgtttctacatgtaatactgatcttttccctccatttccttccgggctttatttttttttctttttctgatgcatttcaggacatttgatgagtcttggagtgtgtttaaatgatgacaagcatgtgatgtgtacactaggtagaccgtacaccctatgaggacaaatacagttctttttttgccatttcatcccctgaacgtgtcacagtacctggcacaaagcacttaaaaatattcatcgaataaataaaatgaatgaaaggatggatggatggattacagacaagtaaaaactcatccatctggaggctgaatgaatgcagatacttcaaaagatctatactttatagtcataatcaataatcactcattttttcaaaggttgtttttattgataaaactcttggttaggtgttgttgaccccacagaaaccaaaagcaactatagtattttgtaattatgccttcctttgtaaaaccagctatcatatagatttttctttgccaggcttatttcattgttgttttgactgaaatggaaatattactggaagctaaaataactcatagacattgggtgaaccataggggagacagtcaggaatggggagatggaaaaaaaacccaaaactcaccagtgcaatcagcaacagatcctccagaagcccattctaagtaatcaaatatgaccgtatgatctaatcaagcagatccaggtagtaggtatctcagctgttgctgtctggtgtgttttaagagacaccagtacagagctcagccctgctccagccgtaggcgatgcccatccaatgaatatagaacacaccatgggaaagagtttcatcagcattggtcccacttctctcaaacaagatgtggtaaggtccaaaaaatgcacccagcatgtcttatgctcattgttctgtcatcttcctgtgcttcctcattgcaaaaccagcattcctctcacggtcagctatgcacaaaatatccttctgttctcctggtcacatcaaagcaccttcacgctatgcagacaggtcattgagggaacggagaaaattaacaaacgcacctaggttatttctattaaaattagcccctcagccggtaggctctgtcagtttccattgaacacaaactctgacaagtctgttgaaaacttttaacctttccaggttgtgtcaacagcttgcaaacacaacaggaggatggtgcctctgagttctgcctttccttttggaatagaggaggtatcagaatttgttaccaccagctttcatgtttatcttcactgctctgctcactccccgctgccacttaaggagcatacaaacaccttactggataaagacaaacatctgtcaattgtctataaggtcctgatgagatttagcttttgcctacttctcccctcatgttttagcccactctcccccactctctactcagctccactgaaggctaccttatggaattcttcaaaaaagcaggtagagttcctcctgccacagggtctttgcatatcctgttccttagcatggagccctcttcttacctagtgatatggtttggctgtgtcccacccaaatctcatcttgaattatagctcccataattcccacatactgt

SEQ ID NO: 15188 - RNA, 16196 nt, Homo sapiens
  source 1..16196: mol_type = other RNA
gctgggattacaggcatgagccactgcacctggtcctggctacattttgtattttttatagagatgggagtctcccaatgttgcccaggctggtcctgagctcttgagctcaagcaatctgcctgcctcagcctcccaaagtgctgggattaaaggtgtgagccaccgcacccagctggaaatttgttagacccctttccgcacttgatgttagacaacagacctataagcaattttatatcttctggcttactttttgtttgttttgctttggtttttgtatttcatggttgggagcaaggcaaaagtgccccaaggttttcggtgtttaagatctccgaagttttaggcccagatcacatatctaatgaatcaaacagacaggacgcaaacccatgcctccgtgacccaaagccccttcatgtataaaatgatgagccagggtcaagctccaggatgcccctgaaagttctagccattcttatggcatagcactgtacactgggacatgacttaatttctccacaggcttctcaaatcctaaaacacgtctctgtccacgcctgaggctcggtatcacaaagccttgtgaaaacgcctctcctgagagaactttcagcccccagacagccgctcattcccttcaagggctgtggtcccaggtcccgggccctagctgtgcttcagtgacatgattcaggagaacctcctccaaagcagcagggcaaaccctgttattttctgggagctgttgtccttgagtcattacctcacactcttagaacttcttccagtttctagagatgaaaatgcgactcagacagtctttgtgactaaggatagaagagaatataagggtgaacacaggacaccttgtggactgaggacataagttcgtaaaagctccctgggctgatgattttaatacaaaagagccaccagacacggttctgagtttaaaagtagaagaaatctggtccagtgtaaatcaagcttattaacgtaaagaattagtgcagaaaaattaaatgagtggatgaagaaaaaagtttggaaggaaaaaataatcctcctcactaccttttaccaaatgagcgttggcaacatgggttggagttgcctttatgcacataatttgccatgcctacattctttcagggcctacaataatgttcctagccatgtatttgaattaaccaggcccagaggataaaactttcaaattaaacacattcctaaaggatttcaggctcattgtgtatgcaccaaggaaacataacatcctaaaaataatacgtacacagagagaagcacattttccatgaacattaaagtggaatatgaattatgacccagctcatgggaatagacatctgattacatgcaaaatggagcttttgtaaataacatcagtcttcgtgagctaccacaattattatcaaccatttaattttattccctagcaactcatccatcgttgttaaaactgtccacttttgttttttaccttctgatgcatgaggctccgaattttataaagttcaccgttaaagctatgtagattaccagcccaacagcgaacgagttcacgaaattattagattcaccaaagcatatgctgcattgtatatctgctattttgggatgtattttgctggtgaattgctagaagcagcaaaattacaacggtagccattctgttcactttttatacaaaggaatcatgaaaatgtgtttaaactttcggtatttgggtatttaagtgcaaagtgactctcaagaaaatcaagtatacttctttctgtctccctggcctgcaatctttgacactattttatgaaataccatccataattccagttggtctatgtcatatataatacgcctgcctcataagtagtaaaataagccactttgtgccttcaccaattctatttcacaacaaagtcaagagacatgtttattaatagaactaaacttttattgatagaagtttaaacaggaatagatgaaggatgctgccaaatgcatcctttgcctgttcctattttaaactcaaaaaccagacacaagaagtacctatggctaatcttttgttctgggagaagttgctaggtggcacctctgaacaatgcctttaacaccttatgggagacctgacctcataaaatacgttgtattttctttcccttgaaattccatttcagtcagaggtgaggattttcattggcttccagaaacctttgagttttaactgcatcaggagtaagcttagaaagcctcctggcttgaagaattttctgaagttagccaagaaaaataagctacgatcaaggaggaaaagctggagtttcagttttctggagattgtacttcctggtaacataaaaacaaaagttaaattcagaaaaattcaactatgaagttagcatcacataaaaaacaatggaaaatatttaactatgcgcatatgtttgtacacaaacagaaatagatataaacagaccttaattagcattgtagactttaattatctttgtacagtaattgggaatggttttgttctgatttattccataatgcttactgtgttctgttaacaactcatttttttccccttccagcccataatagaaggcttttactgcatactttattacatctgcttctcatttaatgaccattgttctggtctgtcagagcgagtggctatacaacttcccaaatctgcaagattaagcaaatattttgacaatgtctagtttcttttttcctttttttcaaaacataccagataaaaataaaaagatttttacttacccacacaacgttaggagagtttttaatctaacgacaataaagaactaagcggcagcaaaatgtacttcatgtggcaaaatacatcaagcaattttctgtcccatttcacttaaaaagtcctaagaatctggtctgaatcacacagctggggttaatgggagcactcctggactgcagggaggttgtgggcccctgggcaaaccacgtggagaccttcaagcttctagaatgagacagaggccttctgctcattttggagggccccggcaggtaagctgaatgataggtgtctgaatcactcactatgaaatgtcatttttaaaaatggtcatgctacatacaaaattgcaataccactgatggcataaggaccagggtcataactctccccaaagaaggtggatacaaatacacaaacagaagcatttctaagcaactgggcagagagatacagagaaaagaggatacagcgaaaaatctattaacccataggcattcattaattctacaaatgatctaatggtgggaagcagaaaatacacaaataaaccaacaaaagcatgacatggacataaatgctaagagggaatggtatgtggaagatgctgcagtcagtggaatgagggaaaggggttaagaacagatgagctttcaagagacagtctatgcctttcagagtagtttaggaaaaaagttaccgaaagataactaggaacagaaaacaaggtgacagaaaggaccgcattaaccccagaagcataagcctcttaaaactttctggtggggagcctctccttggaggcagcaaccagggaaaattcccgcaaggaggtcctacgggagcagccagaattctactagaaagacaggaaagacatgacagggatgggtctgtaggagagcatcggcaaagatagcaagaggatgcaatcctctttagaggaagtagaggtttgccttgttgctattagattgcttcacatctccattggtttgcgtttactatagggcggaaagcacaaagcaggatatgtatgtgcttcaggaagcttaagtgcaaggcaatggggttcatttgtgagctactggcaaaccatttgtatttggggtgggcgtcccgtgcagcacgcctctggaacagtcccttcactgttaacaccactgactgggcccttaattggagcaggtctgcgcgttttaataaacatctttgatgagttctctggactgttccattaaacactcattctaccaaaaatgcctggtaattctctctaaaaatgttttcatgttaccgcttccaggtctttctaaagttaggcagtacaaagaaacaaaaatccaaaagacttgactttaatttagaagtctcaaagagagtgttcaccctagagcagagatttctaaagttgtagtattggactcgcttgcctccacccccacccctgcccttctcccaaaacaagaaaacaaagcagcatcaaagcttgaggtacagaacagaataaaacatgttggtgcagatttgctggcctcggtgaaaacaacctgaatcagtaggtcttggggtatcttcacttttaacaaacactacaggggattttgatgcagtcagttcaggaattaaattttgaaacacacttttgtcaggcggcaacagggtagatagcttaagaatggggtaggaagctagactataggaattcaaatcctagctcctctacttcctagctgtgtgaccttaggaaataaacactctgtgcttcagtctccttatcttcaaaatgggataatgggagcaatgtgtaagaattgaaaaatatgtaaagtacttagtactgtgccagacatgtcgtaagtgcatgaaaaatgttagccactattaacagtggattcatcccaaagtgatttcagctaatgagccaaatttgggtagaggaagtacgctgaagcagattccaaccaaaccaatgaatgaatacagctaagcataaaatagaatccttattaggtatcctcccaccatcatttcagtacggtcagcaccagtctataagctgtacagacatcctatacaatatcaatctcctgtagcacaatatatcctaacaatcctcttgggcacagacgcagccacagggcaggagacaaagcaacagaaccagcaagcacgcactctgctgcctcacttcatgggaatcccattcaacaccagtctaggaagagatgaccttggaatgcagatccagttaattcaattcaatgagcatttattgaacccttgtgatgtatcagagattcacctagatgctgaggataatacaaagagcaacaagaaaatcaccctgtcctcaaggaggtcataatctagtgggaaaaagagatacaagtaattgtaaggcaaggtggcctgagatgaatgctataatagaagatggaagaaggccatgcgaacacagagtaagtagtaattaactctgatgggggcagtcaggaaaggctttcctgaagagcagacatagcatgccattgtgagagatcaataaggcaagcctatgaaattgtttaatgactttatcattcatggaaacaacccagaaaaagcctgagggaccatctctgtctctgcattaacatgggtgtgtttaagatttgattaaatgtttgttgtttctgtaacatcgcatttaaaaaaaaaccaagtatgaacattcgtctattattctgatcttcttcaaagagagaaagagtcctagaaatacttttcttttttccaaagcaaaccctctgcattaatagcaaaagaagaatggcaagttatcgaacgtattatgaactagttagccaaagcgcaagtctgggaaggcccacatttgttttatgtagcaatgagacaaaatatgagagtttttttcttcttatatatggttgcctctttctacttgactataatcattaataatttctttggaccagcagaggaaacaggtattgatcacaataaaacattgcatccacaaacacttgctatagcaggttatggtctccatggaaaccctccaatagaaccaatctgaattcaatttcagaagtaatgagaacagataattttacactcaatcaatcactgtcagctgccgttatcagccaatcagtcattatgtcagtcagtcacactctcaacaaacttcttctgtggcatggtcagatgagaatgttttgacatccagaagcaacacgagaaaattggctcatctttcctggcaagatgccaaagacacagcactgcattgtgtttgctaaggcaataaacagtccaatcaaaatacactgtggtagcggaagattctaggcagcaatttcaataattgttatgatactgatggcagagacgtactttcgacccaaaagtcatacagtttaatcctctcatttaaacatgaagaaacagagcaccagagaagttcaagtatctgcccaaagctgcacagctaactggtggaaagcccacgactaaaacatgagcattctccccttccagtgctcatccaggatgccttgctgctgctcttcactgccttcctttttgaggcaagagggtaaagggatatttgaagattaggttctaattctaaacagagagccccaagcctgtgggagactcacgggatatttgtgaggcttgtgctttggagccaactcaaacctcttgctgtttggggttagctcgtccttggccaagtacaacttctggtttctaaggaggaacaaaagattttgaaacactacagggcaaccaaatcactgttacaaaatgacattttcgataagtttagtgcaggactatcaagaacacatggactgaattccctaaaaatgcttgggagagggaggtaaaatttgaggggaaaaatctggcaaaatacagttgggctcttgtcaacctcaaatgttagaaatgttggcatttgggaattgtgaagaatctgaaaggtgtctggtttctttcttttttctttttactgcattattgctttgtccatttctcagagacagttctctgaggctgaggttcacattcttccttggtaaaacagatggttgggaggccgaggcaggcagatcacgaggtcatgagttcgaggcaggcagatcacgaggtcaggagttcgagaccagcctgaccaacatggtgaaacctgtctctactaagaaaatacaaaaattagctgggtgtggtggtgcacacctgtaatcccagctactcaggaagctgaggcaggcgaatcacttgaacctgggaggtggacgttacagtgagccaagattgcaccactgtactccagcctgggcgacagagtgagactctgtctcaaaaaaaaaaaaaaaaaaatagatggaccagcttgatagtttgcaaacttcaatgtgcatgggaacttaccaaatctgttaaaaatgcaaatccccagatcccacctccagacattttcattcagcaggtgaggctgggcccaggaatctgcctttttaacaaaggacccaggtaattctgatgcactttctttgccaatcagtgttagaaaacattggttaactaatgctatttggtaaagaatttgggccattttgttgatggtagttttccaattacattcctccccaaacattccaacttcgtaaattgtgtgtatcacccatattacaagaacataattctaatggctatgatcacaagctttgatatatatatatatatatatatatatatatatatatatatatatatatataaaatatatgaaatatacattatagtgccactttctattagctgtaagtaggctttatcttaaataggtaggtggtatatgggacactaatacatcccatcagaatttgtctaaggcaaatgaggtgaaaaagcaaagcaagaatatgggttcaggcttgagctaaaactagtaattgcaaaaagaacagtttggaagctttcacatgaaatgcttgcttcatttctctagtctgcttgcctgacctcagctcacgatacctattttatcttctcgcaaaacattgatataaagctttttgcctgtttctacatgtaatactgatcttttccctccatttccttccgggctttatttttttttctttttctgatgcatttcaggacatttgatgagtcttggagtgtgtttaaatgatgacaagcatgtgatgtgtacactaggtagaccgtacaccctatgaggacaaatacagttctttttttgccatttcatcccctgaacgtgtcacagtacctggcacaaagcacttaaaaatattcatcgaataaataaaatgaatgaaaggatggatggatggattacagacaagtaaaaactcatccatctggaggctgaatgaatgcagatacttcaaaagatctatactttatagtcataatcaataatcactcattttttcaaaggttgtttttattgataaaactcttggttaggtgttgttgaccccacagaaaccaaaagcaactatagtattttgtaattatgccttcctttgtaaaaccagctatcatatagatttttctttgccaggcttatttcattgttgttttgactgaaatggaaatattactggaagctaaaataactcatagacattgggtgaaccataggggagacagtcaggaatggggagatggaaaaaaaacccaaaactcaccagtgcaatcagcaacagatcctccagaagcccattctaagtaatcaaatatgaccgtatgatctaatcaagcagatccaggtagtaggtatctcagctgttgctgtctggtgtgttttaagagacaccagtacagagctcagccctgctccagccgtaggcgatgcccatccaatgaatatagaacacaccatgggaaagagtttcatcagcattggtcccacttctctcaaacaagatgtggtaaggtccaaaaaatgcacccagcatgtcttatgctcattgttctgtcatcttcctgtgcttcctcattgcaaaaccagcattcctctcacggtcagctatgcacaaaatatccttctgttctcctggtcacatcaaagcaccttcacgctgagtaactgtgccagtgcagatgggaataacgtaaactccacactattcaaagtgtgctccacgaactgctgccggtcctcaaattggtcattgttggtctggggcaagagaagtacagaaactgagagtaagccttttaaaccttgcccatatatgtgattgtgtaattttgtgtctgttaactctaataataaaaaatggagcttgcatttttaactgcctttttcttttacattgtactttatacaagtattgatccgtcatggactggggggcatggggccagttcttgaccacagaaagtctgagaagccttgctccaggaaaggaaagtagcacagtgccaggaaagagggagagtaggagagtgtgcgcgtttccagcctgggaaagggaagcggaaagcaatctgaaaagcctcccccagggggagtggcatttgagcaaagcctaacaggatggggacggtttggaggcaaagacaggagaaaggacgttttgaggcaaagagaaaggttgaggccaggaagtaaagggtttatgcagggtgccacgcgtatttaacgctctgtgaagcacagagcaggtgagtaataacgataataatagcagctaacatttattgaacacttaccgcaagccaggctctgtgctaagaacatggtgggaattatctcatttgttccttccaactacctgcagggacactgatttgtgaaaatcgttcccagacagacgaaggatattaaataggaggtgagagtgcccctcggggcaatgggcttcaagagcacaggcagacgggagtcagatgccgttcagggacagctgggcaccaactctattgtctgtctcctcctagacgaggatgttgccttactgggcctgagtcaggcttgtcaatgtcctctttaagtggtgggcataatattgtcctgcaagttcttttggaatggtgatgtgagcccaaggacgagaatgaatgggcaggtaaacagaaagcattggcttgccaggtctagcacagcccagccttgctgcagaccttcttcacaaccctggggacagctctgctgggctgtgctgcatctggctcctgctatgggttgccccctggaataggtaagattttgtgcctctggctcattaaatgcagaccttaatctaaccttacaaggtaagtgttctgctctttctagttagtacagaaatgctgcatttgcttttaagtaagtgagaagtgatttgtaaagatgtttcgaactcaggactaactgcctccagagatgcaggaagtaagaccagaacagtaggtgggggccaagacatagatggaggccctgattcccaggcttaggacctgaactttgattctgaggacagcagggaacataaaaatcatatgggagcttctttacctccacaaagaacattctttggctcagcaggacaatatggtgggaaatgacaaagtaactcctgtggccctaggtcaggttctcttgaggaaaacaaaaaggctggaatgatacagctcttcgtaaaccaggtgcctccagtgcctgcggttattcccaagtccacattttgcagacagggccctaaaatgtctagctaggaagttcctgagcctgtttttttaaaattctacacacacacatgcacacacacacgcacgtgtgcacacatgcggatatatacatcctcaccttttcttgagattactgctcagaagaaggcacatttggtttggtctgcttaccagtttgtgaagcacttcagcaccttttaagatgtcaagtgccataaaatcaacgtccttgttatcgtggtaaattgaccttcgttgccaaggcaaagtcagagacagagttaaccatgacagccacgaatagctgttctttgagggccaaaatcatgattttcaatgtttttccatctgaaataggggaacattactcactacagcctataactgtttcctgtcccatgaagctaaattcctacgccagcaatatggtctcaacagaagccctgaaaacagaaatgtcactccgcaaagttcttatttcagccaacaaagctttaagtttagacttaactgtgaaactgaaaatttggctcaccacagagggaactggagagactttttttttaaacaccaggagactgatgtcactgctttgcctatccaatgtcatctcatccctctcccccaaacccaagcaaactctgcagtgagtgacaaacggctgaaatttcagctttacccctcagctagcaggcacttccaaactcatttaatgctcaggtaagttttagctttaaaaaacttggtggggaaaaagaccaggtaatttatcccctattccatgaaaaacaggggagtggggacctatgttaatatgatctttagcagaaaaatgcagtgttgttaggcctggtttctcatacagatttgtttactgtatccatatttactaaaatgtttgttgctgtgactgcaagaaatcagggattaatatttacctctgttacatgaaagaacttactgtcccttttctgcaagtatttggagtcagagattccttaagtaaaaatgctataggccaatgctaaacctgaaaaatggcttagcaagatgctgagttctaacccactctgatgaaattggttatataattggccttgcatcacggatggttatccctatactttgttcttgtcatttcaatcagcccaagcaagtgcactccttctgatttagagacccaaccgatatttgcccacacagacatggtcaggacaacccccagggccttcgtatgttggctcttggcccagacggtataagagtccatttacgacatcaaaatattatgtaaactccctcatcattagagttatgcttttaacctattcatttaaaacgctgactagttatttagcagtgctttaaaaaatatttctaaatcccagaagcaactacatttatgtgaaagatagagcagaacatgttgcgtgtacagtaggcactatttggtggcaggagtctgtggcttcctctacccccagtgaagcctagaggactgcagggatccagcacccacgggtttagagtcttgggtctggtccagtgaagacactgctctctttcatatctccagagtccaccagggagctggctttcgcatcctttaatttggctgcctttactgggaggtgcttcaccatgaaggcttggtaatggatattccaaaaaaaaaaaaatgtaaataggagccacattcaagagcaccatttaaaatgaaaacccacatgaggtctcccagcaaaccactaactttaaagggagcctggctgactaagaagacaggacactggatcctggacatgctgcaccacacagcctgccggccacagccctgcttcttctgaccatggaatttccaaaacagactccctcaaggaaagccaagagcacatttttgtggcattagagtgaagtgaggtttctctttattagagagagatggcattggaaataggctcattttccctcataaggtaccagtctccaaaagactgccttcccggagaagtaccctgggaaggaaaatgcctcagttacggtaccacatggtttgggggactcaagctgtctccaaaaagccctgagaaggaaggatccatttcagcatcacaatttttctgaaccaagcggggatcaacaatgtgggcaccagaactaaatgatccagtaattattctacaaggaggtcccaaagggcccaaaagccatgatgtaatgaacaagaggaggctcagctccagagggcttcctttaggaggtgagtcatgagctgtgtttcgcactggcagagaggaaagctacgtgggtagggcagaaaaaagtgagctgtgtctaggggacaagatgaattggataggtgactcagtgtcaaagatccaccattagtgaaacactgtagaccaggcaatgtaaaggtgtcccataggaacccactgttgatccttcagcacttaaaaaaacaaacaaacaaacaaaaaacaccactgttcttgacgcaggatgaaccattttagcagtgaggggcaagatgaattgggacagcagggagactagctatgaaaatggagtaatcattcaggtgtggtacagatggcattggaatgaagacggtgaatataggaatgcaaattagtaaattaggctcaaccaagagatgactcctgagcaaattatcagacctactgcccaaccgtcagcccagttttaggattttagggttttagacaaaacagtatagggcttggctatgtataccactggcctacagtacaacctattgctaccctacaaataagagaacagcagttaaagacccccacatttcctcttcccctaagcacctcacaacatattcacctatcaccggataccccattcctggaccaagcggccattcctttgaggtgactgattcaacaaggtagtgaaataaagaacttacccagatgattacaaatgccattgaaatgtgacactttcaaattggagagggcatgaagctcaaatgatatgctcattttacggaggaagaagcaaagactgaaaacattgacgagctttcctcaggctctgagagaggtgaactgggtgctgggtgagttctgttcctggctctacccctgaaatactggaagaagctgagagaatttttttttcttttttctgagcctcagattccacatttgtaaatagaaaaaatataactaaatggctcctaggtccctgctagcgctaacttctcgtgtgatcagtgcttctaaaattgcaatgtgtccaggtggggaagttcatttaccccctatctggtttacgctcacttaagggagtgatttctttcctctgaggctctcatcttgcccattattcagagtgagctgcctcctggtgtgctgtcaaaatacatcagcttcaaagacaaacacacacctttcaatcccagtccaagagagtttactgtataatttatgataatgttaagtctgtttctcataaatgttaatggtgctacattttttttcatagatgggtaattctcagaaaagcagctggatgttaaaagttacttttttttttttttttaacataaactgcctcagccaacaaatctgattaaaacaaaactctccaggattgcaaggcacaaagattctgctaatgttagtaagtaaatccaaaaaaaaatcattcaaagattctgttcttataattgtttatctaccatgatttgattaagttcacattcacagacttttctccattttaatgtgtagatattaagaactttttactttaatccaattctttccactcctacaaattgctgaacttgtacattagtattaatataacatgcctaagtacctcccaaagtaaattctttcctgctaaaaatattttgctagcaaatattcggccttttctcatttatagaaactgtaacctttacttcgaagtgccatgcttcatcttttatactctatagaattgttttgactgctaaatgtgtttgaggaattctctcccagacgttagaaagttggattttgaaatcatttgaatctttcaaagttattccctgacgaaagaaaatgcatcaataatttcagattagttactgtactggagcttctgaaattccaaattttctattttgaagcatcaatttgtagaagaatgtaagtattcttaatttttgatgctgtaaaatgcaataacgatagacatattttaacacagaaagataaagacttcaaaagtacataaacagccagaaaaacatacaaaagaattagcttaaacaccttcaaattgcttgggctcaagatacctgggttctaatccctcctccacttgataactctgcaacctcattcattgactcatacatttattcaacaaaggcgtattcggtttgacaccaaggtactgtgctgggcattagttacagagaaatgctagatatggtctctatcctcaaagagcccatagtgtaggggaagaaacagccatgcaaacagatattcctacagtgtggtgggaacattaatacagatatacagagagtattggaaaggaaagagggtaggggtgggggaatgtcagggtttcaagttttcttaaggaaggtgattcctcaactgagccttcaggcctgccctgtctctcggcttgacagggcgcttgtgaggctctcgtaagataaagcccggtaaaggccctgtgaactaaagcacaaaagagctgtactgggattattttccatggtgagaaatagaaaagctacagcataatgagtgagttcttttgcatctctggttattaaggaaaacaaccaaacatgatttggaagagggttttaaaaaattcagtttcagcagattttctcactcttatttgtatgtatagaggacttaaaatgaaaggactatatatctccatttcacagatcaggtcatttaggcacggggccccgagagttaagaaagatggctaggggaaagagaaaaaaaagtctcagccagaggtgagagagagcagctcaggaacctggagccggacggcaatggtgggggatcgcgttttccttctgtgacactctcctcaagggtgacgctacccctgccaaatagggaggaggaatgattttttttttccttcataaaaacaagtcagaaaggaaataaaatccacatttaaaactcccaactgttttttgaaacgagtattttcttcatttcttttccaaggcagacagagcaggtgttaaggctgagttcctcttgtcatgtgaaacaaagatggccctgactaccatgtactgggcgacctataatactgacatcaagcgcaaaaaggaaacaaaaagaaaataaaaaaggaatgcgtgagggtcggagtttttggaagatgaacatgagatgacagcatgagctgggtgttgaagtcgggaagatgcagttaacagaaggggggggggggcgccatggagcagtcgtgtgagccaaggtgcaggaacaagcactcagcttatccagagggaggaccgcttcccagagatattttcaggggcaactttcgcttttttggtttgtttcgtttcttgaggcagggtctcgctttgtcacccaggctggagtacagtggtgcaatcttg

SEQ ID NO: 15189 - RNA, 12599 nt, Homo sapiens
  source 1..12599: mol_type = other RNA
gctgggattacaggcatgagccactgcacctggtcctggctacattttgtattttttatagagatgggagtctcccaatgttgcccaggctggtcctgagctcttgagctcaagcaatctgcctgcctcagcctcccaaagtgctgggattaaaggtgtgagccaccgcacccagctggaaatttgttagacccctttccgcacttgatgttagacaacagacctataagcaattttatatcttctggcttactttttgtttgttttgctttggtttttgtatttcatggttgggagcaaggcaaaagtgccccaaggttttcggtgtttaagatctccgaagttttaggcccagatcacatatctaatgaatcaaacagacaggacgcaaacccatgcctccgtgacccaaagccccttcatgtataaaatgatgagccagggtcaagctccaggatgcccctgaaagttctagccattcttatggcatagcactgtacactgggacatgacttaatttctccacaggcttctcaaatcctaaaacacgtctctgtccacgcctgaggctcggtatcacaaagccttgtgaaaacgcctctcctgagagaactttcagcccccagacagccgctcattcccttcaagggctgtggtcccaggtcccgggccctagctgtgcttcagtgacatgattcaggagaacctcctccaaagcagcagggcaaaccctgttattttctgggagctgttgtccttgagtcattacctcacactcttagaacttcttccagtttctagagatgaaaatgcgactcagacagtctttgtgactaaggatagaagagaatataagggtgaacacaggacaccttgtggactgaggacataagttcgtaaaagctccctgggctgatgattttaatacaaaagagccaccagacacggttctgagtttaaaagtagaagaaatctggtccagtgtaaatcaagcttattaacgtaaagaattagtgcagaaaaattaaatgagtggatgaagaaaaaagtttggaaggaaaaaataatcctcctcactaccttttaccaaatgagcgttggcaacatgggttggagttgcctttatgcacataatttgccatgcctacattctttcagggcctacaataatgttcctagccatgtatttgaattaaccaggcccagaggataaaactttcaaattaaacacattcctaaaggatttcaggctcattgtgtatgcaccaaggaaacataacatcctaaaaataatacgtacacagagagaagcacattttccatgaacattaaagtggaatatgaattatgacccagctcatgggaatagacatctgattacatgcaaaatggagcttttgtaaataacatcagtcttcgtgagctaccacaattattatcaaccatttaattttattccctagcaactcatccatcgttgttaaaactgtccacttttgttttttaccttctgatgcatgaggctccgaattttataaagttcaccgttaaagctatgtagattaccagcccaacagcgaacgagttcacgaaattattagattcaccaaagcatatgctgcattgtatatctgctattttgggatgtattttgctggtgaattgctagaagcagcaaaattacaacggtagccattctgttcactttttatacaaaggaatcatgaaaatgtgtttaaactttcggtatttgggtatttaagtgcaaagtgactctcaagaaaatcaagtatacttctttctgtctccctggcctgcaatctttgacactattttatgaaataccatccataattccagttggtctatgtcatatataatacgcctgcctcataagtagtaaaataagccactttgtgccttcaccaattctatttcacaacaaagtcaagagacatgtttattaatagaactaaacttttattgatagaagtttaaacaggaatagatgaaggatgctgccaaatgcatcctttgcctgttcctattttaaactcaaaaaccagacacaagaagtacctatggctaatcttttgttctgggagaagttgctaggtggcacctctgaacaatgcctttaacaccttatgggagacctgacctcataaaatacgttgtattttctttcccttgaaattccatttcagtcagaggtgaggattttcattggcttccagaaacctttgagttttaactgcatcaggagtaagcttagaaagcctcctggcttgaagaattttctgaagttagccaagaaaaataagctacgatcaaggaggaaaagctggagtttcagttttctggagattgtacttcctggtaacataaaaacaaaagttaaattcagaaaaattcaactatgaagttagcatcacataaaaaacaatggaaaatatttaactatgcgcatatgtttgtacacaaacagaaatagatataaacagaccttaattagcattgtagactttaattatctttgtacagtaattgggaatggttttgttctgatttattccataatgcttactgtgttctgttaacaactcatttttttccccttccagcccataatagaaggcttttactgcatactttattacatctgcttctcatttaatgaccattgttctggtctgtcagagcgagtggctatacaacttcccaaatctgcaagattaagcaaatattttgacaatgtctagtttcttttttcctttttttcaaaacataccagataaaaataaaaagatttttacttacccacacaacgttaggagagtttttaatctaacgacaataaagaactaagcggcagcaaaatgtacttcatgtggcaaaatacatcaagcaattttctgtcccatttcacttaaaaagtcctaagaatctggtctgaatcacacagctggggttaatgggagcactcctggactgcagggaggttgtgggcccctgggcaaaccacgtggagaccttcaagcttctagaatgagacagaggccttctgctcattttggagggccccggcaggtaagctgaatgataggtgtctgaatcactcactatgaaatgtcatttttaaaaatggtcatgctacatacaaaattgcaataccactgatggcataaggaccagggtcataactctccccaaagaaggtggatacaaatacacaaacagaagcatttctaagcaactgggcagagagatacagagaaaagaggatacagcgaaaaatctattaacccataggcattcattaattctacaaatgatctaatggtgggaagcagaaaatacacaaataaaccaacaaaagcatgacatggacataaatgctaagagggaatggtatgtggaagatgctgcagtcagtggaatgagggaaaggggttaagaacagatgagctttcaagagacagtctatgcctttcagagtagtttaggaaaaaagttaccgaaagataactaggaacagaaaacaaggtgacagaaaggaccgcattaaccccagaagcataagcctcttaaaactttctggtggggagcctctccttggaggcagcaaccagggaaaattcccgcaaggaggtcctacgggagcagccagaattctactagaaagacaggaaagacatgacagggatgggtctgtaggagagcatcggcaaagatagcaagaggatgcaatcctctttagaggaagtagaggtttgccttgttgctattagattgcttcacatctccattggtttgcgtttactatagggcggaaagcacaaagcaggatatgtatgtgcttcaggaagcttaagtgcaaggcaatggggttcatttgtgagctactggcaaaccatttgtatttggggtgggcgtcccgtgcagcacgcctctggaacagtcccttcactgttaacaccactgactgggcccttaattggagcaggtctgcgcgttttaataaacatctttgatgagttctctggactgttccattaaacactcattctaccaaaaatgcctggtaattctctctaaaaatgttttcatgttaccgcttccaggtctttctaaagttaggcagtacaaagaaacaaaaatccaaaagacttgactttaatttagaagtctcaaagagagtgttcaccctagagcagagatttctaaagttgtagtattggactcgcttgcctccacccccacccctgcccttctcccaaaacaagaaaacaaagcagcatcaaagcttgaggtacagaacagaataaaacatgttggtgcagatttgctggcctcggtgaaaacaacctgaatcagtaggtcttggggtatcttcacttttaacaaacactacaggggattttgatgcagtcagttcaggaattaaattttgaaacacacttttgtcaggcggcaacagggtagatagcttaagaatggggtaggaagctagactataggaattcaaatcctagctcctctacttcctagctgtgtgaccttaggaaataaacactctgtgcttcagtctccttatcttcaaaatgggataatgggagcaatgtgtaagaattgaaaaatatgtaaagtacttagtactgtgccagacatgtcgtaagtgcatgaaaaatgttagccactattaacagtggattcatcccaaagtgatttcagctaatgagccaaatttgggtagaggaagtacgctgaagcagattccaaccaaaccaatgaatgaatacagctaagcataaaatagaatccttattaggtatcctcccaccatcatttcagtacggtcagcaccagtctataagctgtacagacatcctatacaatatcaatctcctgtagcacaatatatcctaacaatcctcttgggcacagacgcagccacagggcaggagacaaagcaacagaaccagcaagcacgcactctgctgcctcacttcatgggaatcccattcaacaccagtctaggaagagatgaccttggaatgcagatccagttaattcaattcaatgagcatttattgaacccttgtgatgtatcagagattcacctagatgctgaggataatacaaagagcaacaagaaaatcaccctgtcctcaaggaggtcataatctagtgggaaaaagagatacaagtaattgtaaggcaaggtggcctgagatgaatgctataatagaagatggaagaaggccatgcgaacacagagtaagtagtaattaactctgatgggggcagtcaggaaaggctttcctgaagagcagacatagcatgccattgtgagagatcaataaggcaagcctatgaaattgtttaatgactttatcattcatggaaacaacccagaaaaagcctgagggaccatctctgtctctgcattaacatgggtgtgtttaagatttgattaaatgtttgttgtttctgtaacatcgcatttaaaaaaaaaccaagtatgaacattcgtctattattctgatcttcttcaaagagagaaagagtcctagaaatacttttcttttttccaaagcaaaccctctgcattaatagcaaaagaagaatggcaagttatcgaacgtattatgaactagttagccaaagcgcaagtctgggaaggcccacatttgttttatgtagcaatgagacaaaatatgagagtttttttcttcttatatatggttgcctctttctacttgactataatcattaataatttctttggaccagcagaggaaacaggtattgatcacaataaaacattgcatccacaaacacttgctatagcaggttatggtctccatggaaaccctccaatagaaccaatctgaattcaatttcagaagtaatgagaacagataattttacactcaatcaatcactgtcagctgccgttatcagccaatcagtcattatgtcagtcagtcacactctcaacaaacttcttctgtggcatggtcagatgagaatgttttgacatccagaagcaacacgagaaaattggctcatctttcctggcaagatgccaaagacacagcactgcattgtgtttgctaaggcaataaacagtccaatcaaaatacactgtggtagcggaagattctaggcagcaatttcaataattgttatgatactgatggcagagacgtactttcgacccaaaagtcatacagtttaatcctctcatttaaacatgaagaaacagagcaccagagaagttcaagtatctgcccaaagctgcacagctaactggtggaaagcccacgactaaaacatgagcattctccccttccagtgctcatccaggatgccttgctgctgctcttcactgccttcctttttgaggcaagagggtaaagggatatttgaagattaggttctaattctaaacagagagccccaagcctgtgggagactcacgggatatttgtgaggcttgtgctttggagccaactcaaacctcttgctgtttggggttagctcgtccttggccaagtacaacttctggtttctaaggaggaacaaaagattttgaaacactacagggcaaccaaatcactgttacaaaatgacattttcgataagtttagtgcaggactatcaagaacacatggactgaattccctaaaaatgcttgggagagggaggtaaaatttgaggggaaaaatctggcaaaatacagttgggctcttgtcaacctcaaatgttagaaatgttggcatttgggaattgtgaagaatctgaaaggtgtctggtttctttcttttttctttttactgcattattgctttgtccatttctcagagacagttctctgaggctgaggttcacattcttccttggtaaaacagatggttgggaggccgaggcaggcagatcacgaggtcatgagttcgaggcaggcagatcacgaggtcaggagttcgagaccagcctgaccaacatggtgaaacctgtctctactaagaaaatacaaaaattagctgggtgtggtggtgcacacctgtaatcccagctactcaggaagctgaggcaggcgaatcacttgaacctgggaggtggacgttacagtgagccaagattgcaccactgtactccagcctgggcgacagagtgagactctgtctcaaaaaaaaaaaaaaaaaaatagatggaccagcttgatagtttgcaaacttcaatgtgcatgggaacttaccaaatctgttaaaaatgcaaatccccagatcccacctccagacattttcattcagcaggtgaggctgggcccaggaatctgcctttttaacaaaggacccaggtaattctgatgcactttctttgccaatcagtgttagaaaacattggttaactaatgctatttggtaaagaatttgggccattttgttgatggtagttttccaattacattcctccccaaacattccaacttcgtaaattgtgtgtatcacccatattacaagaacataattctaatggctatgatcacaagctttgatatatatatatatatatatatatatatatatatatatatatatatatataaaatatatgaaatatacattatagtgccactttctattagctgtaagtaggctttatcttaaataggtaggtggtatatgggacactaatacatcccatcagaatttgtctaaggcaaatgaggtgaaaaagcaaagcaagaatatgggttcaggcttgagctaaaactagtaattgcaaaaagaacagtttggaagctttcacatgaaatgcttgcttcatttctctagtctgcttgcctgacctcagctcacgatacctattttatcttctcgcaaaacattgatataaagctttttgcctgtttctacatgtaatactgatcttttccctccatttccttccgggctttatttttttttctttttctgatgcatttcaggacatttgatgagtcttggagtgtgtttaaatgatgacaagcatgtgatgtgtacactaggtagaccgtacaccctatgaggacaaatacagttctttttttgccatttcatcccctgaacgtgtcacagtacctggcacaaagcacttaaaaatattcatcgaataaataaaatgaatgaaaggatggatggatggattacagacaagtaaaaactcatccatctggaggctgaatgaatgcagatacttcaaaagatctatactttatagtcataatcaataatcactcattttttcaaaggttgtttttattgataaaactcttggttaggtgttgttgaccccacagaaaccaaaagcaactatagtattttgtaattatgccttcctttgtaaaaccagctatcatatagatttttctttgccaggcttatttcattgttgttttgactgaaatggaaatattactggaagctaaaataactcatagacattgggtgaaccataggggagacagtcaggaatggggagatggaaaaaaaacccaaaactcaccagtgcaatcagcaacagatcctccagaagcctgtaaaaattaagacaacttttaaaactctctttgcctgtcatcactacacacatcccaggctcacagtctttctgcatcatgcagatgacagaggtaacccttaggaagcttaacttatctcactggtaggtttcacagcctcatgccagtgacgtcacagaaaacaactttaaatcttccatgaaacaagcaaactggaggagagatgaattcaatgagctatcagaggtgctttccatcctattagaaaaaaggaggaaagcaggaaggaaggcagtaagaaaaggaggagaaattaacatttgtcgagcatccattgacaaccaggcgccacactaaactcttcatattttatctcatttgaagcttattatatttccagggggtggaaattcattggttcattttattttattcatttatttactttatttattttagagacagctctcactttgtcatccaggctggagtgcactggcacaatcatagctcactgcagcctcgaactcctgggcttaagggatcttcctgcctcacattcccaaagtgctggaattacaggcgcgagccaccatgcccagctagtatgttcattttatagatgagggaaatagggctcagagaggttcatccccatgccccaacagctaatgaacaataaagctgggactaaagtaatagcaaatatttactaaggacttaacgtcagtcagtttcatgtgtgttaactattaattcattgaatcctccttttaatcttatgaggtaggtacctctatgcccttttcagaggtcacagaacaaacacagagaggttaaataacttgcccaaggagtcacagctgatacatagcagagctggggctggaacctgcgtgatcagcatcagaccctcgtctcttaactaccacactcagccattctctacaatagcgtctaggttggcctttttccaaaggctaaatcctttccggaatacaactttgattttatgtttctagagaaaacaaaaaaggcatacctcaacaatagcctattagacttttccaagcatgacaaatcatgtgtatttgttatatatacagataggctatgtggtcttaattaaggtgaccatataatttattgtccaaaccatgaaagaaggtgctatcaataattatccagggacaacagtggtaacctggaactgttccaagatggcaagggtgcctggtcaccctagtcctaatgaataaatacacacacacacacatacacacaaacacacaaacacacaattagatatcgttactttcagacacattctgatactacccgctggagtacggatgtgtagttaaatgctttctaacactgtgtgagcccaccctcctcccacctcaagagctgctagccctttctttacctaatgcatttcttttaacttgttttctcacaaaagactgtacgtaattggtcagccatgagagattaatttgtgcttagctggctgagcggacacaagataactcaatagcggatgatgccagtgcatgaaccagcagcttctctcgataagccttcctacctactcgggacctcgtccctccatagcctgcttctttgggaattgccagccaagtcctttactttatttacctcatttttgcctgcctggagaaattcaaacttgcagtttttaagtttcttcatgggccatttttcttacggaaatagaaacagtagcaaagacacccagactctccccttctaaagcaatgcatcaaagagtgcactggggtatgtggatagcagagaaactgagcaagggcaagtttatgcatatccttcatcctgctcacattgtttataactgcagtcagacacagacagcaggctgagagtgatggacatggcgatgacaatggcgatgatggtgatgggaagacttctaagaacttaaaaagcgttttacacagatgatctcatctaatgctatctcagccctaggtggtgggtgcaattatcattcccattttagagatggaaaaacagatatttacagagggcaaacattctgccccacgtccaatctaggtaacttaacctcagagctaacactctaacccacagggcctggacattcaaatgcacaagtcaaccacagatgacagagtacaggacaaattggactggagagatccatgcctcccaactcctcatctcacagatgagaactccagttcagtccttttgcctcctccagaaaatacttacctgtcaagaactttgtaaaaatgaaatgagagaaggttaaaaacataaccaagaagtgctacataaatgttttctactgtcactagaccagcccttaaacgctatttcagaatgtattactctaatagagtaatttttaaatacctggacatcagagctaattggacatcagacattggagctaattccacctaaccatagaaatgcactgtggcctgggtttatgcctgtcatacagttccctcccacggcaggtacatttgccacatcccaatacactgccagtaaagataaagtaccttctaatatacttataaaagcacagagtgcaggggctagggactatagaagaaggcaggaggcaaggaagcaaagggttttatttttttttaatgtccccaactcctctaacctggtccctttgctttgtttggctggtacgacaggtggtgactcttaagcactgtgtagcctgctcttgtgtccagattatcccaagcagtctgaaacttcaagagaatttgcagtaatgcacaagtcaggatttggttcccagagcaaagctgtgctcaaaggattggacatcagaaacaaacctaaaaagagccacaaacacggaccccaggctcctcccaccccctccctaactcacctgtagggtttaaagagattccattttaatgaagcaggatgggcataacacttgggaaggaaaggaaatctggcctaccccaaagcaattagcttcctctgctaggaagagactgtgcttgtgtcctgaggtttttatttcatttttcctcaaggggatgggaagttcgctggtctaagattcatgcctttcagactgctcctcaagtgaggaggccacgtggccctgtaacccaaatgccaggcccttggtatcaccttctgctcctctcagagacaccttgatgtcaccttccgctcctctcagagtcactctgccgagtcgccctgtgatgaggacattatctggacctgtgctaatacagtggctaccagccacctgtggccaccgagcacttgaacctggccagtcccaactgaaatgtgctgtcagtgcaaaatccacacctgagttggaagtgaataaaaatatctcaatttttttacatgaattacacattaaaattgtactattttggatatattgagttaaaaaatgtatctccaaaattaattccacctttttcttttcaattcttaaaaaacatggtcacacaaatatttaacactgtgtctgtgcttatcatatatacgctatatttccactggacagcactgttctagacactcatcaggtatgattgctccatttcccagcagcatgtgtatcaaccaggagcctgctagaaatacagaatctcaggccccatcccagacctactgaatcataatctgcattttcagagatccccaggtaatctgcatgcacattaaagtctgtgaagcactgccctggggtctaaaacattacttggcacacaagaggcacttgagaaatatttgttgaatgaataaatgagttatgtctaggaagctgctgtacttgggggcactcgggaaaatgtgaagggctgtccctggctttctccttagctcagttaatattgatatactcatcagattaatcacctttcattttagtagctgatacggtttggctgtgtctccacccacatctcatcttgaattgtagctcccataattcccacatgtccaggga

SEQ ID NO: 15190 - RNA, 3464 nt, Homo sapiens
  source 1..3464: mol_type = other RNA
gctgggattacaggcatgagccactgcacctggtcctggctacattttgtattttttatagagatgggagtctcccaatgttgcccaggctggtcctgagctcttgagctcaagcaatctgcctgcctcagcctcccaaagtgctgggattaaaggtgtgagccaccgcacccagctggaaatttgttagacccctttccgcacttgatgttagacaacagacctataagcaattttatatcttctggcttactttttgtttgttttgctttggtttttgtatttcatggttgggagcaaggcaaaagtgccccaaggttttcggtgtttaagatctccgaagttttaggcccagatcacatatctaatgaatcaaacagacaggacgcaaacccatgcctccgtgacccaaagccccttcatgtataaaatgatgagccagggtcaagctccaggatgcccctgaaagttctagccattcttatggcatagcactgtacactgggacatgacttaatttctccacaggcttctcaaatcctaaaacacgtctctgtccacgcctgaggctcggtatcacaaagccttgtgaaaacgcctctcctgagagaactttcagcccccagacagccgctcattcccttcaagggctgtggtcccaggtcccgggccctagctgtgcttcagtgacatgattcaggagaacctcctccaaagcagcagggcaaaccctgttattttctgggagctgttgtccttgagtcattacctcacactcttagaacttcttccagtttctagagatgaaaatgcgactcagacagtctttgtgactaaggatagaagagaatataagggtgaacacaggacaccttgtggactgaggacataagttcgtaaaagctccctgggctgatgattttaatacaaaagagccaccagacacggttctgagtttaaaagtagaagaaatctggtccagtgtaaatcaagcttattaacgtaaagaattagtgcagaaaaattaaatgagtggatgaagaaaaaagtttggaaggaaaaaataatcctcctcactaccttttaccaaatgagcgttggcaacatgggttggagttgcctttatgcacataatttgccatgcctacattctttcagggcctacaataatgttcctagccatgtatttgaattaaccaggcccagaggataaaactttcaaattaaacacattcctaaaggatttcaggctcattgtgtatgcaccaaggaaacataacatcctaaaaataatacgtacacagagagaagcacattttccatgaacattaaagtggaatatgaattatgacccagctcatgggaatagacatctgattacatgcaaaatggagcttttgtaaataacatcagtcttcgtgagctaccacaattattatcaaccatttaattttattccctagcaactcatccatcgttgttaaaactgtccacttttgttttttaccttctgatgcatgaggctccgaattttataaagttcaccgttaaagctatgtagattaccagcccaacagcgaacgagttcacgaaattattagattcaccaaagcatatgctgcattgtatatctgctattttgggatgtattttgctggtgaattgctagaagcagcaaaattacaacggtagccattctgttcactttttatacaaaggaatcatgaaaatgtgtttaaactttcggtatttgggtatttaagtgcaaagtgactctcaagaaaatcaagtatacttctttctgtctccctggcctgcaatctttgacactattttatgaaataccatccataattccagttggtctatgtcatatataatacgcctgcctcataagtagtaaaataagccactttgtgccttcaccaattctatttcacaacaaagtcaagagacatgtttattaatagaactaaacttttattgatagaagtttaaacaggaatagatgaaggatgctgccaaatgcatcctttgcctgttcctattttaaactcaaaaaccagacacaagaagtacctatggctaatcttttgttctgggagaagttgctaggtggcacctctgaacaatgcctttaacaccttatgggagacctgacctcataaaatacgttgtattttctttcccttgaaattccatttcagtcagaggtgaggattttcattggcttccagaaacctttgagttttaactgcatcaggagtaagcttagaaagcctcctggcttgaagaattttctgaagttagccaagaaaaataagctacgatcaaggaggaaaagctggagtttcagttttctggagattgtacttcgggatatttgtgaggcttgtgctttggagccaactcaaacctcttgctgtttggggttagctcgtccttggccaagtacaacttctggtttcagtgcaatcagcaacagatcctccagaagcccattctaagtaatcaaatatgaccgtatgatctaatcaagcagatccaggtagtaggtatctcagctgttgctgtctggtgtgttttaagagacaccagtacagagctcagccctgctccagccgtaggcgatgcccatccaatgaatatagaacacaccatgggaaagagtttcatcagcattggtcccacttctctcaaacaagatgtggtaaggtccaaaaaatgcacccagcatgtcttatgctcattgttctgtcatcttcctgtgcttcctcattgcaaaaccagcattcctctcacggtcagctatgcacaaaatatccttctgttctcctggtcacatcaaagcaccttcacgctatgcagacaggtcattgagggaacggagaaaattaacaaacgcacctaggttatttctattaaaattagcccctcagccggtaggctctgtcagtttccattgaacacaaactctgacaagtctgttgaaaacttttaacctttccaggttgtgtcaacagcttgcaaacacaacaggaggatggtgcctctgagttctgcctttccttttggaatagaggaggtatcagaatttgttaccaccagctttcatgtttatcttcactgctctgctcactccccgctgccacttaaggagcatacaaacaccttactggataaagacaaacatctgtcaattgtctataaggtcctgatgagatttagcttttgcctacttctcccctcatgttttagcccactctcccccactctctactcagctccactgaaggctaccttatggaattcttcaaaaaagcaggtagagttcctcctgccacagggtctttgcatatcctgttccttagcatggagccctcttcttacctagtgatatggtttggctgtgtcccacccaaatctcatcttgaattatagctcccataattcccacatactgt

SEQ ID NO: 15191 - RNA, 3742 nt, Homo sapiens
  source 1..3742: mol_type = other RNA
gctgggattacaggcatgagccactgcacctggtggaattgggatcttgaattacagcttctagtttaaacagcatgtggtgtttcagagggaggaccatggagagctacatgtcatgttaggaaagaattaacagacagaggtagtatatattaagggaatgaaccactctaaacactgaatatcactggcaaccctaaaatgatgaggatttaatgacttgcacactcaagtgaaccaagggataaaactcctacaaaaagaaaatactgtaagtattaatgctaggttatcatcaagaactaatggtttaattttgcactggatttgtattctttccaggcctggacatgatattttaaaggctggttttgtctagaggaggatggccaagatgtgacaggtaagaaaagcatgccatatgaggaatgacttaaaggactagagtaacagcagctcaaagtaagactgagggggagaccacccactgcacatatctcaagtgccgttaaagagttgcagatagtagatctggactacaaggagaatccacaggcagacttcagctgatatgaggaaaaactctctcgttattagagttgcccaacttttgagtaataaatgcatagccaccagaggctacctgaccatgcccatgggtgaaagctgtggtagcaggggtccctgtgacacaataatagaaagctggacctaatgacctctgggtcttgccactctaaacttccatgactctcatcaatgggttgaaagtacttcattccattaaacctctattaagtgccatttcccctattaatttctaagaaagtaaatctctctgctaaatctaaccactggaaataatcaaattcaccactattctcacagcccagtaggctgctatcttccatcttctttgtcacaatgttgcaagtggcctcagatacttgactttcgccatatgtgtctttccagcctgcttccacttcctagtccatctctcaacaatctcccctccccacctctcattcctccttgcactgacttcatttctcattagaagcaggtgtcagggcgaagagaggaaaacaaggtcaaggaagtgaggcagaatggagtattcagagcccaaattttcttataaagaaaatcactttgaagggggaagataagtgggagacgaaaacaatgagctgacacttatgccatagtctaccttccagggagcaggcagtggtgctgccaccaaggcaccagagtgatgattttcttgtctccagaataatgacttcccacaatggccaaagacaactgaggtcaggtgctctgtcctagcttttataccattgagtgagggggtggggaagggaaaaatataaaaggatagaaaggaaaggaataaatgaagccagggccatttgcgccttggagaaatggctaggtatgagggaggaataagggttaaaactagttagggagattactgggtgttgacagaaaaaataaaagtcagttcctgagaggtgaagaagaatagagcgcctcaatgcagtcactgtcaccttggatgctaaccattccagagggcatctgatgatcaattcaacatcctgctgtttctcttggcaccccaatcaggatcctggagtggctaccacaagactcacctatatcagaggacactgggttaatgtaaaaagctgaaggatactgattagggtagaagtcttacatgtttggaccaaatccaatgtggacaaagtagctgagcagcaggaagttgaggggtccacagctgagcctggtgtactccccagagcattctccagatggctcgaattaccacaatcatgcttcaattaaaactgtcataaaacttgggataggggtttggaagaacagggcattgaaagtgcagagaaaatgtagagtgtatagaggtgactgaagagggtgatagaaagaagtgtccttccaccaaaacatccatttcttttggttggaaggcaaggactggaaaagaggggtgggggcagcaaatgctgtccctttctttcctcataaatctggagcctagcctacttggacagtttgctgatgactctgatgagggcaccattttcatctttcagcctctggttgtcggatttcagttctgttaacacctggagtagtggaggagggaagtgagttggagagtaggggcaagaactagagctcctgggtgtccgaggactcgatggactccgagagtctggccaccactcgggtcagggccctgttctcagcctgcagttgctcgttcatctgcttcaaggtttgaatctgttttagctggtggaggttcttcatttcttcctccatttctgacattttgcgctccaaggctcgcctctcccgtttctccatctccagcactgatgatcggtcagaggtcttttcttgtttctgctgggccaccttctcaagcttggactttatatctgctagctctagctgggcttcctgaagttttgttttcagtttttggttttcagtcagagcactctcatagagttttttataatctctgttgctgtcttcttctacacggctggtcagggtggctaggcgggcctcccgggcctcccgacgggctcttgctgaagcccggtcaccgtaagaatcactggttgtaggattactacctcccgattccaacctagaaagtctttcatgccacgtttctttgacctcttcagagccatcagtttcatcctcatcctttgtccagaaattgatgcctgtgcctcttcgtcgttccttgggccgcctcctctctcggatggacagcctcttagaggactgctcatccaaatctgcttcttcattctcatttttgtccatttcctttgcagttgtagtgtttgtggtagtctctgaactctcagaatcagggactgaaaatctatttgtccatagcaggtgggaactggtgtagagtgagggtcttgacgtagaaggagatgctggcgtggtgggtttgtctggctgagctgggcacctcaggcgatgacagataggctcttcatccagactcctgccccagggctgctggccctccccagcttctgttgctggaactgctgagggctcatgcttctcagggctcccctcaagcccttcagtgtctgtgggcttctcacgaggctgctcctgagcttgcctctctgccctcgaccggctgaatgtcctttctgcttcttgaaggtctgttagggtgacaccttgagtagaccttcgtgtctgccgagcttgtctggagcgtgctttccgtaaagactctgcttcctcatcccgtacaggagtcagataggacctgctgcttctgacattccaggcccagcacttgctgatgtctcaactcagcacactggagttagcatccaaacacagagtactaacaaactatggcagaggcttgtctcaattccccagaacacccagatcaacttcctgtgcctctgatttccataaaaccaggaatggcaaggaactctattgccagatcaaatcattccaggtgaaagcaggtcaagctatctcagacacaccttgccacacacttgtgcagcaactttcccagaagcccaattttcaacaaacaggtggccactcctctgactgtccttctctaaacactggagcccattttatgagattgtaccagcaactgtccttttctaacatgggaaaatcaact

SEQ ID NO: 15192 - RNA, 3617 nt, Homo sapiens
  source 1..3617: mol_type = other RNA
gctgggattacaggcatgagccactgcacctggtggaattgggatcttgaattacagcttctagtttaaacagcatgtggtgtttcagagggaggaccatggagagctacatgtcatgttaggaaagaattaacagacagaggtagtatatattaagggaatgaaccactctaaacactgaatatcactggcaaccctaaaatgatgaggatttaatgacttgcacactcaagtgaaccaagggataaaactcctacaaaaagaaaatactgtaagtattaatgctaggttatcatcaagaactaatggtttaattttgcactggatttgtattctttccaggcctggacatgatattttaaaggctggttttgtctagaggaggatggccaagatgtgacaggtaagaaaagcatgccatatgaggaatgacttaaaggactagagtaacagcagctcaaagtaagactgagggggagaccacccactgcacatatctcaagtgccgttaaagagttgcagatagtagatctggactacaaggagaatccacaggcagacttcagctgatatgaggaaaaactctctcgttattagagttgcccaacttttgagtaataaatgcatagccaccagaggctacctgaccatgcccatgggtgaaagctgtggtagcaggggtccctgtgacacaataatagaaagctggacctaatgacctctgggtcttgccactctaaacttccatgactctcatcaatgggttgaaagtacttcattccattaaacctctattaagtgccatttcccctattaatttctaagaaagtaaatctctctgctaaatctaaccactggaaataatcaaattcaccactattctcacagcccagtaggctgctatcttccatcttctttgtcacaatgttgcaagtggcctcagatacttgactttcgccatatgtgtctttccagcctgcttccacttcctagtccatctctcaacaatctcccctccccacctctcattcctccttgcactgacttcatttctcattagaagcaggtgtcagggcgaagagaggaaaacaaggtcaaggaagtgaggcagaatggagtattcagagcccaaattttcttataaagaaaatcactttgaagggggaagataagtgggagacgaaaacaatgagctgacacttatgccatagtctaccttccagggagcaggcagtggtgctgccaccaaggcaccagagtgatgattttcttgtctccagaataatgacttcccacaatggccaaagacaactgaggtcaggtgctctgtcctagcttttataccattgagtgagggggtggggaagggaaaaatataaaaggatagaaaggaaaggaataaatgaagccagggccatttgcgccttggagaaatggctaggtatgagggaggaataagggttaaaactagttagggagattactgggtgttgacagaaaaaataaaagtcagttcctgagaggtgaagaagaatagagcgcctcaatgcagtcactgtcaccttggatgctaaccattccagagggcatctgatgatcaattcaacatcctgctgtttctcttggcaccccaatcaggatcctggagtggctaccacaagactcacctatatcagaggacactgggttaatgtaaaaagctgaaggatactgattagggtagaagtcttacatgtttggaccaaatccaatgtggacaaagtagctgagcagcaggaagttgaggggtccacagctgagcctggtgtactccccagagcattctccagatggctcgaattaccacaatcatgcttcaattaaaactgtcataaaacttgggataggggtttggaagaacagggcattgaaagtgcagagaaaatgtagagtgtatagaggtgactgaagagggtgatagaaagaagtgtccttccaccaaaacatccatttcttttggttggaaggcaaggactggaaaagaggggtgggggcagcaaatgctgtccctttctttcctcataaatctggagcctagcctacttggacagtttgctgatgactctgatgagggcaccattttcatctttcagcctctggttgtcggatttcagttctgttaacaccttcatttcttcctccatttctgacattttgcgctccaaggctcgcctctcccgtttctccatctccagcactgatgatcggtcagaggtcttttcttgtttctgctgggccaccttctcaagcttggactttatatctgctagctctagctgggcttcctgaagttttgttttcagtttttggttttcagtcagagcactctcatagagttttttataatctctgttgctgtcttcttctacacggctggtcagggtggctaggcgggcctcccgggcctcccgacgggctcttgctgaagcccggtcaccgtaagaatcactggttgtaggattactacctcccgattccaacctagaaagtctttcatgccacgtttctttgacctcttcagagccatcagtttcatcctcatcctttgtccagaaattgatgcctgtgcctcttcgtcgttccttgggccgcctcctctctcggatggacagcctcttagaggactgctcatccaaatctgcttcttcattctcatttttgtccatttcctttgcagttgtagtgtttgtggtagtctctgaactctcagaatcagggactgaaaatctatttgtccatagcaggtgggaactggtgtagagtgagggtcttgacgtagaaggagatgctggcgtggtgggtttgtctggctgagctgggcacctcaggcgatgacagataggctcttcatccagactcctgccccagggctgctggccctccccagcttctgttgctggaactgctgagggctcatgcttctcagggctcccctcaagcccttcagtgtctgtgggcttctcacgaggctgctcctgagcttgcctctctgccctcgaccggctgaatgtcctttctgcttcttgaaggtctgttagggtgacaccttgagtagaccttcgtgtctgccgagcttgtctggagcgtgctttccgtaaagactctgcttcctcatcccgtacaggagtcagataggacctcctcttctccctggcttccacagaggaatctgttccagtaatggagagcacaggagtagctgtaaccccattggcagtgctaggaagagggcgattggtgatcacacagagcggggtgctagaagagacattgtctgctgttttctctgctgttgtgtcggcctgggatttgtgaggagtcctgccatgatgtacagatgcagtagtgtttgcactgattggtgcagggcaagaagaggcaggttgccactggctgccccgagaggtagatgaaccaatggtaatgggtgaggtagcaggagatgaattgcgattggctgaaatgtagggacttgtggggtcactacttctaccaaatgaagcacttctctgcaccaaacttgcgagtttcacatcttgatggatcttttcaagtaagttgatacataggtggaggga

SEQ ID NO: 15193 - RNA, 5363 nt, Homo sapiens
  source 1..5363: mol_type = other RNA
gctgggattacaggcatgagccactgcacctggtggaattgggatcttgaattacagcttctagtttaaacagcatgtggtgtttcagagggaggaccatggagagctacatgtcatgttaggaaagaattaacagacagaggtagtatatattaagggaatgaaccactctaaacactgaatatcactggcaaccctaaaatgatgaggatttaatgacttgcacactcaagtgaaccaagggataaaactcctacaaaaagaaaatactgtaagtattaatgctaggttatcatcaagaactaatggtttaattttgcactggatttgtattctttccaggcctggacatgatattttaaaggctggttttgtctagaggaggatggccaagatgtgacaggtaagaaaagcatgccatatgaggaatgacttaaaggactagagtaacagcagctcaaagtaagactgagggggagaccacccactgcacatatctcaagtgccgttaaagagttgcagatagtagatctggactacaaggagaatccacaggcagacttcagctgatatgaggaaaaactctctcgttattagagttgcccaacttttgagtaataaatgcatagccaccagaggctacctgaccatgcccatgggtgaaagctgtggtagcaggggtccctgtgacacaataatagaaagctggacctaatgacctctgggtcttgccactctaaacttccatgactctcatcaatgggttgaaagtacttcattccattaaacctctattaagtgccatttcccctattaatttctaagaaagtaaatctctctgctaaatctaaccactggaaataatcaaattcaccactattctcacagcccagtaggctgctatcttccatcttctttgtcacaatgttgcaagtggcctcagatacttgactttcgccatatgtgtctttccagcctgcttccacttcctagtccatctctcaacaatctcccctccccacctctcattcctccttgcactgacttcatttctcattagaagcaggtgtcagggcgaagagaggaaaacaaggtcaaggaagtgaggcagaatggagtattcagagcccaaattttcttataaagaaaatcactttgaagggggaagataagtgggagacgaaaacaatgagctgacacttatgccatagtctaccttccagggagcaggcagtggtgctgccaccaaggcaccagagtgatgattttcttgtctccagaataatgacttcccacaatggccaaagacaactgaggtcaggtgctctgtcctagcttttataccattgagtgagggggtggggaagggaaaaatataaaaggatagaaaggaaaggaataaatgaagccagggccatttgcgccttggagaaatggctaggtatgagggaggaataagggttaaaactagttagggagattactgggtgttgacagaaaaaataaaagtcagttcctgagaggtgaagaagaatagagcgcctcaatgcagtcactgtcaccttggatgctaaccattccagagggcatctgatgatcaattcaacatcctgctgtttctcttggcaccccaatcaggatcctggagtggctaccacaagactcacctatatcagaggacactgggttaatgtaaaaagctgaaggatactgattagggtagaagtcttacatgtttggaccaaatccaatgtggacaaagtagctgagcagcaggaagttgaggggtccacagctgagcctggtgtactccccagagcattctccagatggctcgaattaccacaatcatgcttcaattaaaactgtcataaaacttgggataggggtttggaagaacagggcattgaaagtgcagagaaaatgtagagtgtatagaggtgactgaagagggtgatagaaagaagtgtccttccaccaaaacatccatttcttttggttggaaggcaaggactggaaaagaggggtgggggcagcaaatgctgtccctttctttcctcataaatctggagcctagcctacttggacagtttgctgatgactctgatgagggcaccattttcatctttcagcctctggttgtcggatttcagttctgttaacaccttcatttcttcctccatttctgacattttgcgctccaaggctcgcctctcccgtttctccatctccagcactgatgatcggtcagaggtcttttcttgtttctgctgggccaccttctcaagcttggactttatatctgctagctctagctgggcttcctgaagttttgttttcagtttttggttttcagtcagagcactctcatagagttttttataatctctgttgctgtcttcttctacacggctggtcagggtggctaggcgggcctcccgggcctcccgacgggctcttgctgaagcccggtcaccgtaagaatcactggttgtaggattactacctcccgattccaacctagaaagtctttcatgccacgtttctttgacctcttcagagccatcagtttcatcctcatcctttgtccagaaattgatgcctgtgcctcttcgtcgttccttgggccgcctcctctctcggatggacagcctcttagaggactgctcatccaaatctgcttcttcattctcatttttgtccatttcctttgcagttgtagtgtttgtggtagtctctgaactctcagaatcagggactgaaaatctatttgtccatagcaggtgggaactggtgtagagtgagggtcttgacgtagaaggagatgctggcgtggtgggtttgtctggctgagctgggcacctcaggcgatgacagataggctcttcatccagactcctgccccagggctgctggccctccccagcttctgttgctggaactgctgagggctcatgcttctcagggctcccctcaagcccttcagtgtctgtgggcttctcacgaggctgctcctgagcttgcctctctgccctcgaccggctgaatgtcctttctgcttcttgaaggtctgttagggtgacaccttgagtagaccttcgtgtctgccgagcttgtctggagcgtgctttccgtaaagactctgcttcctcatcccgtacaggagtcagataggacctcctcttctccctggcttccacagaggaatctgttccagtaatggagagcacaggagtagctgtaaccccattggcagtgctaggaagagggcgattggtgatcacacagagcggggtgctagaagagacattgtctgctgttttctctgctgttgtgtcggcctgggatttgtgaggagtcctgccatgatgtacagatgcagtagtgtttgcactgattggtgcagggcaagaagaggcaggttgccactggctgccccgagaggtagatgaaccaatggtaatgggtgaggtagcaggagatgaattgcgattggctgaaatgtagggacttgtggggtcactacttctaccaaatgaagcacttttcaagtaagttgatacataggtggagggagcaattgtctgtgggatttcatttccttttgcttcatccctccatagctgccgggtataggagccactcctcactagattaacagctgattctctgttctccttttcttcaatatcacttgtgctgttgagcttccggggtgctagtgaactaatatagcttttgttttctctctccttatctttgttgtccagtagagcagaaatccgagggcttgaagaggagcgatagatggaagagcctcggtcccttataggttccctggaattggccacctcactcagcatgttgtggctgccagtttttctcagtcccaatctccatgaagaaggagattcatctttgggctcttctggcttgttaaaaaggccagaagagaacctcctagcagaagaggcagagaaggtattttgagctggtgctggtatctgctctgtgatactactcttgctttcagagttggaatgattgacaaaggcttctggctttttatctgcctccttctcagtttctgactcagaagcttcatcttcaccttcctcctcctctgagctggagctactagattctttattttcttcctccatttcttgggacttaggtgtctcctcctcatagagcatcttctctttgttcttaaagaacccactctgaatcttgctgttcagatctgactcaatgagtttattccgtgtctccttttcacttcgaagcacattctgcttcttctggagcaactccaaatgctccacgagaccctcatcagccacatcaaatggtgtctggcccagtttatttcgaatatccatgtcacaaagtgcttctgccaggatggagcaagcctccttcactccccagtgtgcagcagcatggaggggagtccagccatcataatcctgaacattgagttcatagccagcctgaattaaaagtctgaggacttcagagtagcccttggcagcagccacatgaagggctgtagcccctgagcgagcctgcctcacatcctctattttcccactgttgagccactggcgggcatcctgcaacatctgctgctcttcttcttttcttgactgctctagatcaactccttgcttctttacttgctccagaagaagatccttcatggctggctcttctgcaaggtcagagggaacttcaccttcactattgacaatacctacactggctccgtgattaatgaaatactctgctatgttgagatagccacaggaagctgctgcatgaaggggtgtccagccctcgttgtcttgctggtttacattggctctgttctccaccagaaacttcaccatgtccaaattttcatcaatacatgcctggtgcagggctgtcaagccgtccacgttgaccgtgttgatatcagcacctcttgccagaagctttctcacctcgtcggtgtccccgctagagcaggcggccagaaagacagcaccgtcctcgaagcggaccctggggctcccgcgcctggtcagcggctgccgccccgcgcctcgtcgctccgcaggctcctgctctgtcagcgagccccgccagcgccgaagctgctctgcccgccgcattcgcgccgactctgcccgcttccctcctaggtgctccagttccgccattgctccggcctcggcagctgctgccaaaactaccaacactaaattactgttggggctcgagttgccgctgccgcctctctcagagcgcttcagcccggagcagagggcggagaccctcgcgccgccatctttactcctcccgccagtagtacc

SEQ ID NO: 15194 - RNA, 5234 nt, Homo sapiens
  source 1..5234: mol_type = other RNA
gctgggattacaggcatgagccactgcacctggtggaattgggatcttgaattacagcttctagtttaaacagcatgtggtgtttcagagggaggaccatggagagctacatgtcatgttaggaaagaattaacagacagaggtagtatatattaagggaatgaaccactctaaacactgaatatcactggcaaccctaaaatgatgaggatttaatgacttgcacactcaagtgaaccaagggataaaactcctacaaaaagaaaatactgtaagtattaatgctaggttatcatcaagaactaatggtttaattttgcactggatttgtattctttccaggcctggacatgatattttaaaggctggttttgtctagaggaggatggccaagatgtgacaggtaagaaaagcatgccatatgaggaatgacttaaaggactagagtaacagcagctcaaagtaagactgagggggagaccacccactgcacatatctcaagtgccgttaaagagttgcagatagtagatctggactacaaggagaatccacaggcagacttcagctgatatgaggaaaaactctctcgttattagagttgcccaacttttgagtaataaatgcatagccaccagaggctacctgaccatgcccatgggtgaaagctgtggtagcaggggtccctgtgacacaataatagaaagctggacctaatgacctctgggtcttgccactctaaacttccatgactctcatcaatgggttgaaagtacttcattccattaaacctctattaagtgccatttcccctattaatttctaagaaagtaaatctctctgctaaatctaaccactggaaataatcaaattcaccactattctcacagcccagtaggctgctatcttccatcttctttgtcacaatgttgcaagtggcctcagatacttgactttcgccatatgtgtctttccagcctgcttccacttcctagtccatctctcaacaatctcccctccccacctctcattcctccttgcactgacttcatttctcattagaagcaggtgtcagggcgaagagaggaaaacaaggtcaaggaagtgaggcagaatggagtattcagagcccaaattttcttataaagaaaatcactttgaagggggaagataagtgggagacgaaaacaatgagctgacacttatgccatagtctaccttccagggagcaggcagtggtgctgccaccaaggcaccagagtgatgattttcttgtctccagaataatgacttcccacaatggccaaagacaactgaggtcaggtgctctgtcctagcttttataccattgagtgagggggtggggaagggaaaaatataaaaggatagaaaggaaaggaataaatgaagccagggccatttgcgccttggagaaatggctaggtatgagggaggaataagggttaaaactagttagggagattactgggtgttgacagaaaaaataaaagtcagttcctgagaggtgaagaagaatagagcgcctcaatgcagtcactgtcaccttggatgctaaccattccagagggcatctgatgatcaattcaacatcctgctgtttctcttggcaccccaatcaggatcctggagtggctaccacaagactcacctatatcagaggacactgggttaatgtaaaaagctgaaggatactgattagggtagaagtcttacatgtttggaccaaatccaatgtggacaaagtagctgagcagcaggaagttgaggggtccacagctgagcctggtgtactccccagagcattctccagatggctcgaattaccacaatcatgcttcaattaaaactgtcataaaacttgggataggggtttggaagaacagggcattgaaagtgcagagaaaatgtagagtgtatagaggtgactgaagagggtgatagaaagaagtgtccttccaccaaaacatccatttcttttggttggaaggcaaggactggaaaagaggggtgggggcagcaaatgctgtccctttctttcctcataaatctggagcctagcctacttggacagtttgctgatgactctgatgagggcaccattttcatctttcagcctctggttgtcggatttcagttctgttaacaccttcatttcttcctccatttctgacattttgcgctccaaggctcgcctctcccgtttctccatctccagcactgatgatcggtcagaggtcttttcttgtttctgctgggccaccttctcaagcttggactttatatctgctagctctagctgggcttcctgaagttttgttttcagtttttggttttcagtcagagcactctcatagagttttttataatctctgttgctgtcttcttctacacggctggtcagggtggctaggcgggcctcccgggcctcccgacgggctcttgctgaagcccggtcaccgtaagaatcactggttgtaggattactacctcccgattccaacctagaaagtctttcatgccacgtttctttgacctcttcagagccatcagtttcatcctcatcctttgtccagaaattgatgcctgtgcctcttcgtcgttccttgggccgcctcctctctcggatggacagcctcttagaggactgctcatccaaatctgcttcttcattctcatttttgtccatttcctttgcagttgtagtgtttgtggtagtctctgaactctcagaatcagggactgaaaatctatttgtccatagcaggtgggaactggtgtagagtgagggtcttgacgtagaaggagatgctggcgtggtgggtttgtctggctgagctgggcacctcaggcgatgacagataggctcttcatccagactcctgccccagggctgctggccctccccagcttctgttgctggaactgctgagggctcatgcttctcagggctcccctcaagcccttcagtgtctgtgggcttctcacgaggctgctcctgagcttgcctctctgccctcgaccggctgaatgtcctttctgcttcttgaaggtctgttagggtgacaccttgagtagaccttcgtgtctgccgagcttgtctggagcgtgctttccgtaaagactctgcttcctcatcccgtacaggagtcagataggacctcctcttctccctggcttccacagaggaatctgttccagtaatggagagcacaggagtagctgtaaccccattggcagtgctaggaagagggcgattggtgatcacacagagcggggtgctagaagagacattgtctgctgttttctctgctgttgtgtcggcctgggatttgtgaggagtccttttcaagtaagttgatacataggtggagggagcaattgtctgtgggatttcatttccttttgcttcatccctccatagctgccgggtataggagccactcctcactagattaacagctgattctctgttctccttttcttcaatatcacttgtgctgttgagcttccggggtgctagtgaactaatatagcttttgttttctctctccttatctttgttgtccagtagagcagaaatccgagggcttgaagaggagcgatagatggaagagcctcggtcccttataggttccctggaattggccacctcactcagcatgttgtggctgccagtttttctcagtcccaatctccatgaagaaggagattcatctttgggctcttctggcttgttaaaaaggccagaagagaacctcctagcagaagaggcagagaaggtattttgagctggtgctggtatctgctctgtgatactactcttgctttcagagttggaatgattgacaaaggcttctggctttttatctgcctccttctcagtttctgactcagaagcttcatcttcaccttcctcctcctctgagctggagctactagattctttattttcttcctccatttcttgggacttaggtgtctcctcctcatagagcatcttctctttgttcttaaagaacccactctgaatcttgctgttcagatctgactcaatgagtttattccgtgtctccttttcacttcgaagcacattctgcttcttctggagcaactccaaatgctccacgagaccctcatcagccacatcaaatggtgtctggcccagtttatttcgaatatccatgtcacaaagtgcttctgccaggatggagcaagcctccttcactccccagtgtgcagcagcatggaggggagtccagccatcataatcctgaacattgagttcatagccagcctgaattaaaagtctgaggacttcagagtagcccttggcagcagccacatgaagggctgtagcccctgagcgagcctgcctcacatcctctattttcccactgttgagccactggcgggcatcctgcaacatctgctgctcttcttcttttcttgactgctctagatcaactccaggattaaatcatcaggttaaatattatgtgatacagatccattaagggaatgcaccttgcttctttacttgctccagaagaagatccttcatggctggctcttctgcaaggtcagagggaacttcaccttcactattgacaatacctacactggctccgtgattaatgaaatactctgctatgttgagatagccacaggaagctgctgcatgaaggggtgtccagccctcgttgtcttgctggtttacattggctctgttctccaccagaaacttcaccatgtccaaattttcatcaatacatgcctggtgcagggctgtcaagccgtccacgttgaccgtgttgatatcagcacctcttgccagaagctttctcacctcgtcggtgtccccgctagagcaggcggccagaaagacagcaccgtcctcgaagcggaccctggggctcccgcgcctggtcagcggctgccgccccgcgcctcgtcgctccgcaggctcctgctctgtcagcgagccccgccagcgccgaagctgctctgcccgccgcattcgcgccgactctgcccgcttccctcctaggtgctccagttccgccattgctccggcctcggcagctgctgccaaaactaccaacactaaattactgttggggctcgagttgccgctgccgcctctctcagagcgcttcagcccggagcagagggcggagaccctcgcgccgccatctttactcctcccgccagtagt

SEQ ID NO: 15195 - RNA, 5180 nt, Homo sapiens
  source 1..5180: mol_type = other RNA
gctgggattacaggcatgagccactgcacctggtggaattgggatcttgaattacagcttctagtttaaacagcatgtggtgtttcagagggaggaccatggagagctacatgtcatgttaggaaagaattaacagacagaggtagtatatattaagggaatgaaccactctaaacactgaatatcactggcaaccctaaaatgatgaggatttaatgacttgcacactcaagtgaaccaagggataaaactcctacaaaaagaaaatactgtaagtattaatgctaggttatcatcaagaactaatggtttaattttgcactggatttgtattctttccaggcctggacatgatattttaaaggctggttttgtctagaggaggatggccaagatgtgacaggtaagaaaagcatgccatatgaggaatgacttaaaggactagagtaacagcagctcaaagtaagactgagggggagaccacccactgcacatatctcaagtgccgttaaagagttgcagatagtagatctggactacaaggagaatccacaggcagacttcagctgatatgaggaaaaactctctcgttattagagttgcccaacttttgagtaataaatgcatagccaccagaggctacctgaccatgcccatgggtgaaagctgtggtagcaggggtccctgtgacacaataatagaaagctggacctaatgacctctgggtcttgccactctaaacttccatgactctcatcaatgggttgaaagtacttcattccattaaacctctattaagtgccatttcccctattaatttctaagaaagtaaatctctctgctaaatctaaccactggaaataatcaaattcaccactattctcacagcccagtaggctgctatcttccatcttctttgtcacaatgttgcaagtggcctcagatacttgactttcgccatatgtgtctttccagcctgcttccacttcctagtccatctctcaacaatctcccctccccacctctcattcctccttgcactgacttcatttctcattagaagcaggtgtcagggcgaagagaggaaaacaaggtcaaggaagtgaggcagaatggagtattcagagcccaaattttcttataaagaaaatcactttgaagggggaagataagtgggagacgaaaacaatgagctgacacttatgccatagtctaccttccagggagcaggcagtggtgctgccaccaaggcaccagagtgatgattttcttgtctccagaataatgacttcccacaatggccaaagacaactgaggtcaggtgctctgtcctagcttttataccattgagtgagggggtggggaagggaaaaatataaaaggatagaaaggaaaggaataaatgaagccagggccatttgcgccttggagaaatggctaggtatgagggaggaataagggttaaaactagttagggagattactgggtgttgacagaaaaaataaaagtcagttcctgagaggtgaagaagaatagagcgcctcaatgcagtcactgtcaccttggatgctaaccattccagagggcatctgatgatcaattcaacatcctgctgtttctcttggcaccccaatcaggatcctggagtggctaccacaagactcacctatatcagaggacactgggttaatgtaaaaagctgaaggatactgattagggtagaagtcttacatgtttggaccaaatccaatgtggacaaagtagctgagcagcaggaagttgaggggtccacagctgagcctggtgtactccccagagcattctccagatggctcgaattaccacaatcatgcttcaattaaaactgtcataaaacttgggataggggtttggaagaacagggcattgaaagtgcagagaaaatgtagagtgtatagaggtgactgaagagggtgatagaaagaagtgtccttccaccaaaacatccatttcttttggttggaaggcaaggactggaaaagaggggtgggggcagcaaatgctgtccctttctttcctcataaatctggagcctagcctacttggacagtttgctgatgactctgatgagggcaccattttcatctttcagcctctggttgtcggatttcagttctgttaacaccttcatttcttcctccatttctgacattttgcgctccaaggctcgcctctcccgtttctccatctccagcactgatgatcggtcagaggtcttttcttgtttctgctgggccaccttctcaagcttggactttatatctgctagctctagctgggcttcctgaagttttgttttcagtttttggttttcagtcagagcactctcatagagttttttataatctctgttgctgtcttcttctacacggctggtcagggtggctaggcgggcctcccgggcctcccgacgggctcttgctgaagcccggtcaccgtaagaatcactggttgtaggattactacctcccgattccaacctagaaagtctttcatgccacgtttctttgacctcttcagagccatcagtttcatcctcatcctttgtccagaaattgatgcctgtgcctcttcgtcgttccttgggccgcctcctctctcggatggacagcctcttagaggactgctcatccaaatctgcttcttcattctcatttttgtccatttcctttgcagttgtagtgtttgtggtagtctctgaactctcagaatcagggactgaaaatctatttgtccatagcaggtgggaactggtgtagagtgagggtcttgacgtagaaggagatgctggcgtggtgggtttgtctggctgagctgggcacctcaggcgatgacagataggctcttcatccagactcctgccccagggctgctggccctccccagcttctgttgctggaactgctgagggctcatgcttctcagggctcccctcaagcccttcagtgtctgtgggcttctcacgaggctgctcctgagcttgcctctctgccctcgaccggctgaatgtcctttctgcttcttgaaggtctgttagggtgacaccttgagtagaccttcgtgtctgccgagcttgtctggagcgtgctttccgtaaagactctgcttcctcatcccgtacaggagtcagataggacctcctcttctccctggcttccacagaggaatctgttccagtaatggagagcacaggagtagctgtaaccccattggcagtgctaggaagagggcgattggtgatcacacagagcggggtgctagaagagacattgtctgctgttttctctgctgttgtgtcggcctgggatttgtgaggagtccttttcaagtaagttgatacataggtggagggagcaattgtctgtgggatttcatttccttttgcttcatccctccatagctgccgggtataggagccactcctcactagattaacagctgattctctgttctccttttcttcaatatcacttgtgctgttgagcttccggggtgctagtgaactaatatagcttttgttttctctctccttatctttgttgtccagtagagcagaaatccgagggcttgaagaggagcgatagatggaagagcctcggtcccttataggttccctggaattggccacctcactcagcatgttgtggctgccagtttttctcagtcccaatctccatgaagaaggagattcatctttgggctcttctggcttgttaaaaaggccagaagagaacctcctagcagaagaggcagagaaggtattttgagctggtgctggtatctgctctgtgatactactcttgctttcagagttggaatgattgacaaaggcttctggctttttatctgcctccttctcagtttctgactcagaagcttcatcttcaccttcctcctcctctgagctggagctactagattctttattttcttcctccatttcttgggacttaggtgtctcctcctcatagagcatcttctctttgttcttaaagaacccactctgaatcttgctgttcagatctgactcaatgagtttattccgtgtctccttttcacttcgaagcacattctgcttcttctggagcaactccaaatgctccacgagaccctcatcagccacatcaaatggtgtctggcccagtttatttcgaatatccatgtcacaaagtgcttctgccaggatggagcaagcctccttcactccccagtgtgcagcagcatggaggggagtccagccatcataatcctgaacattgagttcatagccagcctgaattaaaagtctgaggacttcagagtagcccttggcagcagccacatgaagggctgtagcccctgagcgagcctgcctcacatcctctattttcccactgttgagccactggcgggcatcctgcaacatctgctgctcttcttcttttcttgactgctctagatcaactccttgcttctttacttgctccagaagaagatccttcatggctggctcttctgcaaggtcagagggaacttcaccttcactattgacaatacctacactggctccgtgattaatgaaatactctgctatgttgagatagccacaggaagctgctgcatgaaggggtgtccagccctcgttgtcttgctggtttacattggctctgttctccaccagaaacttcaccatgtccaaattttcatcaatacatgcctggtgcagggctgtcaagccgtccacgttgaccgtgttgatatcagcacctcttgccagaagctttctcacctcgtcggtgtccccgctagagcaggcggccagaaagacagcaccgtcctcgaagcggaccctggggctcccgcgcctggtcagcggctgccgccccgcgcctcgtcgctccgcaggctcctgctctgtcagcgagccccgccagcgccgaagctgctctgcccgccgcattcgcgccgactctgcccgcttccctcctaggtgctccagttccgccattgctccggcctcggcagctgctgccaaaactaccaacactaaattactgttggggctcgagttgccgctgccgcctctctcagagcgcttcagcccggagcagagggcggagaccctcgcgccgccatctttactcctcccgccagtagtacc

SEQ ID NO: 15196 - RNA, 3561 nt, Homo sapiens
  source 1..3561: mol_type = other RNA
gctgggattacaggcatgagccactgcacctggtggaattgggatcttgaattacagcttctagtttaaacagcatgtggtgtttcagagggaggaccatggagagctacatgtcatgttaggaaagaattaacagacagaggtagtatatattaagggaatgaaccactctaaacactgaatatcactggcaaccctaaaatgatgaggatttaatgacttgcacactcaagtgaaccaagggataaaactcctacaaaaagaaaatactgtaagtattaatgctaggttatcatcaagaactaatggtttaattttgcactggatttgtattctttccaggcctggacatgatattttaaaggctggttttgtctagaggaggatggccaagatgtgacaggtaagaaaagcatgccatatgaggaatgacttaaaggactagagtaacagcagctcaaagtaagactgagggggagaccacccactgcacatatctcaagtgccgttaaagagttgcagatagtagatctggactacaaggagaatccacaggcagacttcagctgatatgaggaaaaactctctcgttattagagttgcccaacttttgagtaataaatgcatagccaccagaggctacctgaccatgcccatgggtgaaagctgtggtagcaggggtccctgtgacacaataatagaaagctggacctaatgacctctgggtcttgccactctaaacttccatgactctcatcaatgggttgaaagtacttcattccattaaacctctattaagtgccatttcccctattaatttctaagaaagtaaatctctctgctaaatctaaccactggaaataatcaaattcaccactattctcacagcccagtaggctgctatcttccatcttctttgtcacaatgttgcaagtggcctcagatacttgactttcgccatatgtgtctttccagcctgcttccacttcctagtccatctctcaacaatctcccctccccacctctcattcctccttgcactgacttcatttctcattagaagcaggtgtcagggcgaagagaggaaaacaaggtcaaggaagtgaggcagaatggagtattcagagcccaaattttcttataaagaaaatcactttgaagggggaagataagtgggagacgaaaacaatgagctgacacttatgccatagtctaccttccagggagcaggcagtggtgctgccaccaaggcaccagagtgatgattttcttgtctccagaataatgacttcccacaatggccaaagacaactgaggtcaggtgctctgtcctagcttttataccattgagtgagggggtggggaagggaaaaatataaaaggatagaaaggaaaggaataaatgaagccagggccatttgcgccttggagaaatggctaggtatgagggaggaataagggttaaaactagttagggagattactgggtgttgacagaaaaaataaaagtcagttcctgagaggtgaagaagaatagagcgcctcaatgcagtcactgtcaccttggatgctaaccattccagagggcatctgatgatcaattcaacatcctgctgtttctcttggcaccccaatcaggatcctggagtggctaccacaagactcacctatatcagaggacactgggttaatgtaaaaagctgaaggatactgattagggtagaagtcttacatgtttggaccaaatccaatgtggacaaagtagctgagcagcaggaagttgaggggtccacagctgagcctggtgtactccccagagcattctccagatggctcgaattaccacaatcatgcttcaattaaaactgtcataaaacttgggataggggtttggaagaacagggcattgaaagtgcagagaaaatgtagagtgtatagaggtgactgaagagggtgatagaaagaagtgtccttccaccaaaacatccatttcttttggttggaaggcaaggactggaaaagaggggtgggggcagcaaatgctgtccctttctttcctcataaatctggagcctagcctacttggacagtttgctgatgactctgatgagggcaccattttcatctttcagcctctggttgtcggatttcagttctgttaacaccttcatttcttcctccatttctgacattttgcgctccaaggctcgcctctcccgtttctccatctccagcactgatgatcggtcagaggtcttttcttgtttctgctgggccaccttctcaagcttggactttatatctgctagctctagctgggcttcctgaagttttgttttcagtttttggttttcagtcagagcactctcatagagttttttataatctctgttgctgtcttcttctacacggctggtcagggtggctaggcgggcctcccgggcctcccgacgggctcttgctgaagcccggtcaccgtaagaatcactggttgtaggattactacctcccgattccaacctagaaagtctttcatgccacgtttctttgacctcttcagagccatcagtttcatcctcatcctttgtccagaaattgatgcctgtgcctcttcgtcgttccttgggccgcctcctctctcggatggacagcctcttagaggactgctcatccaaatctgcttcttcattctcatttttgtccatttcctttgcagttgtagtgtttgtggtagtctctgaactctcagaatcagggactgaaaatctatttgtccatagcaggtgggaactggtgtagagtgagggtcttgacgtagaaggagatgctggcgtggtgggtttgtctggctgagctgggcacctcaggcgatgacagataggctcttcatccagactcctgccccagggctgctggccctccccagcttctgttgctggaactgctgagggctcatgcttctcagggctcccctcaagcccttcagtgtctgtgggcttctcacgaggctgctcctgagcttgcctctctgccctcgaccggctgaatgtcctttctgcttcttgaaggtctgttagggtgacaccttgagtagaccttcgtgtctgccgagcttgtctggagcgtgctttccgtaaagactctgcttcctcatcccgtacaggagtcagataggacctgctgcttctgacattccaggcccagcacttgctgatgtctcaactcagcacactggagttagcatccaaacacagagtactaacaaactatggcagaggcttgtctcaattccccagaacacccagatcaacttcctgtgcctctgatttccataaaaccaggaatggcaaggaactctattgccagatcaaatcattccaggtgaaagcaggtcaagctatctcagacacaccttgccacacacttgtgcagcaactttcccagaagcccaattttcaacaaacaggtggccactcctctgactgtccttctctaaacactggagcccattttatgagattgtaccagcaactgtccttttctaacatgggaaaatcaact

SEQ ID NO: 15197 - RNA, 5504 nt, Homo sapiens
  source 1..5504: mol_type = other RNA
gctgggattacaggcatgagccactgcacctggtggaattgggatcttgaattacagcttctagtttaaacagcatgtggtgtttcagagggaggaccatggagagctacatgtcatgttaggaaagaattaacagacagaggtagtatatattaagggaatgaaccactctaaacactgaatatcactggcaaccctaaaatgatgaggatttaatgacttgcacactcaagtgaaccaagggataaaactcctacaaaaagaaaatactgtaagtattaatgctaggttatcatcaagaactaatggtttaattttgcactggatttgtattctttccaggcctggacatgatattttaaaggctggttttgtctagaggaggatggccaagatgtgacaggtaagaaaagcatgccatatgaggaatgacttaaaggactagagtaacagcagctcaaagtaagactgagggggagaccacccactgcacatatctcaagtgccgttaaagagttgcagatagtagatctggactacaaggagaatccacaggcagacttcagctgatatgaggaaaaactctctcgttattagagttgcccaacttttgagtaataaatgcatagccaccagaggctacctgaccatgcccatgggtgaaagctgtggtagcaggggtccctgtgacacaataatagaaagctggacctaatgacctctgggtcttgccactctaaacttccatgactctcatcaatgggttgaaagtacttcattccattaaacctctattaagtgccatttcccctattaatttctaagaaagtaaatctctctgctaaatctaaccactggaaataatcaaattcaccactattctcacagcccagtaggctgctatcttccatcttctttgtcacaatgttgcaagtggcctcagatacttgactttcgccatatgtgtctttccagcctgcttccacttcctagtccatctctcaacaatctcccctccccacctctcattcctccttgcactgacttcatttctcattagaagcaggtgtcagggcgaagagaggaaaacaaggtcaaggaagtgaggcagaatggagtattcagagcccaaattttcttataaagaaaatcactttgaagggggaagataagtgggagacgaaaacaatgagctgacacttatgccatagtctaccttccagggagcaggcagtggtgctgccaccaaggcaccagagtgatgattttcttgtctccagaataatgacttcccacaatggccaaagacaactgaggtcaggtgctctgtcctagcttttataccattgagtgagggggtggggaagggaaaaatataaaaggatagaaaggaaaggaataaatgaagccagggccatttgcgccttggagaaatggctaggtatgagggaggaataagggttaaaactagttagggagattactgggtgttgacagaaaaaataaaagtcagttcctgagaggtgaagaagaatagagcgcctcaatgcagtcactgtcaccttggatgctaaccattccagagggcatctgatgatcaattcaacatcctgctgtttctcttggcaccccaatcaggatcctggagtggctaccacaagactcacctatatcagaggacactgggttaatgtaaaaagctgaaggatactgattagggtagaagtcttacatgtttggaccaaatccaatgtggacaaagtagctgagcagcaggaagttgaggggtccacagctgagcctggtgtactccccagagcattctccagatggctcgaattaccacaatcatgcttcaattaaaactgtcataaaacttgggataggggtttggaagaacagggcattgaaagtgcagagaaaatgtagagtgtatagaggtgactgaagagggtgatagaaagaagtgtccttccaccaaaacatccatttcttttggttggaaggcaaggactggaaaagaggggtgggggcagcaaatgctgtccctttctttcctcataaatctggagcctagcctacttggacagtttgctgatgactctgatgagggcaccattttcatctttcagcctctggttgtcggatttcagttctgttaacaccttcatttcttcctccatttctgacattttgcgctccaaggctcgcctctcccgtttctccatctccagcactgatgatcggtcagaggtcttttcttgtttctgctgggccaccttctcaagcttggactttatatctgctagctctagctgggcttcctgaagttttgttttcagtttttggttttcagtcagagcactctcatagagttttttataatctctgttgctgtcttcttctacacggctggtcagggtggctaggcgggcctcccgggcctcccgacgggctcttgctgaagcccggtcaccgtaagaatcactggttgtaggattactacctcccgattccaacctagaaagtctttcatgctatgtcaaggacagcagaagaatgctgatgctctacccactgaatcttgatactctgagtaggcttttaagttgtccttcaagaagacgttccttcactcaaggaggtgagatgctactagcaagtcaattcgaacatgtaacccacgtttctttgacctcttcagagccatcagtttcatcctcatcctttgtccagaaattgatgcctgtgcctcttcgtcgttccttgggccgcctcctctctcggatggacagcctcttagaggactgctcatccaaatctgcttcttcattctcatttttgtccatttcctttgcagttgtagtgtttgtggtagtctctgaactctcagaatcagggactgaaaatctatttgtccatagcaggtgggaactggtgtagagtgagggtcttgacgtagaaggagatgctggcgtggtgggtttgtctggctgagctgggcacctcaggcgatgacagataggctcttcatccagactcctgccccagggctgctggccctccccagcttctgttgctggaactgctgagggctcatgcttctcagggctcccctcaagcccttcagtgtctgtgggcttctcacgaggctgctcctgagcttgcctctctgccctcgaccggctgaatgtcctttctgcttcttgaaggtctgttagggtgacaccttgagtagaccttcgtgtctgccgagcttgtctggagcgtgctttccgtaaagactctgcttcctcatcccgtacaggagtcagataggacctcctcttctccctggcttccacagaggaatctgttccagtaatggagagcacaggagtagctgtaaccccattggcagtgctaggaagagggcgattggtgatcacacagagcggggtgctagaagagacattgtctgctgttttctctgctgttgtgtcggcctgggatttgtgaggagtcctgccatgatgtacagatgcagtagtgtttgcactgattggtgcagggcaagaagaggcaggttgccactggctgccccgagaggtagatgaaccaatggtaatgggtgaggtagcaggagatgaattgcgattggctgaaatgtagggacttgtggggtcactacttctaccaaatgaagcacttttcaagtaagttgatacataggtggagggagcaattgtctgtgggatttcatttccttttgcttcatccctccatagctgccgggtataggagccactcctcactagattaacagctgattctctgttctccttttcttcaatatcacttgtgctgttgagcttccggggtgctagtgaactaatatagcttttgttttctctctccttatctttgttgtccagtagagcagaaatccgagggcttgaagaggagcgatagatggaagagcctcggtcccttataggttccctggaattggccacctcactcagcatgttgtggctgccagtttttctcagtcccaatctccatgaagaaggagattcatctttgggctcttctggcttgttaaaaaggccagaagagaacctcctagcagaagaggcagagaaggtattttgagctggtgctggtatctgctctgtgatactactcttgctttcagagttggaatgattgacaaaggcttctggctttttatctgcctccttctcagtttctgactcagaagcttcatcttcaccttcctcctcctctgagctggagctactagattctttattttcttcctccatttcttgggacttaggtgtctcctcctcatagagcatcttctctttgttcttaaagaacccactctgaatcttgctgttcagatctgactcaatgagtttattccgtgtctccttttcacttcgaagcacattctgcttcttctggagcaactccaaatgctccacgagaccctcatcagccacatcaaatggtgtctggcccagtttatttcgaatatccatgtcacaaagtgcttctgccaggatggagcaagcctccttcactccccagtgtgcagcagcatggaggggagtccagccatcataatcctgaacattgagttcatagccagcctgaattaaaagtctgaggacttcagagtagcccttggcagcagccacatgaagggctgtagcccctgagcgagcctgcctcacatcctctattttcccactgttgagccactggcgggcatcctgcaacatctgctgctcttcttcttttcttgactgctctagatcaactccttgcttctttacttgctccagaagaagatccttcatggctggctcttctgcaaggtcagagggaacttcaccttcactattgacaatacctacactggctccgtgattaatgaaatactctgctatgttgagatagccacaggaagctgctgcatgaaggggtgtccagccctcgttgtcttgctggtttacattggctctgttctccaccagaaacttcaccatgtccaaattttcatcaatacatgcctggtgcagggctgtcaagccgtccacgttgaccgtgttgatatcagcacctcttgccagaagctttctcacctcgtcggtgtccccgctagagcaggcggccagaaagacagcaccgtcctcgaagcggaccctggggctcccgcgcctggtcagcggctgccgccccgcgcctcgtcgctccgcaggctcctgctctgtcagcgagccccgccagcgccgaagctgctctgcccgccgcattcgcgccgactctgcccgcttccctcctaggtgctccagttccgccattgctccggcctcggcagctgctgccaaaactaccaacactaaattactgttggggctcgagttgccgctgccgcctctctcagagcgcttcagcccggagcagagggcggagaccctcgcgccgccatctttactcctcccgccagtagt

SEQ ID NO: 15198 - RNA, 5321 nt, Homo sapiens
  source 1..5321: mol_type = other RNA
gctgggattacaggcatgagccactgcacctggtggaattgggatcttgaattacagcttctagtttaaacagcatgtggtgtttcagagggaggaccatggagagctacatgtcatgttaggaaagaattaacagacagaggtagtatatattaagggaatgaaccactctaaacactgaatatcactggcaaccctaaaatgatgaggatttaatgacttgcacactcaagtgaaccaagggataaaactcctacaaaaagaaaatactgtaagtattaatgctaggttatcatcaagaactaatggtttaattttgcactggatttgtattctttccaggcctggacatgatattttaaaggctggttttgtctagaggaggatggccaagatgtgacaggtaagaaaagcatgccatatgaggaatgacttaaaggactagagtaacagcagctcaaagtaagactgagggggagaccacccactgcacatatctcaagtgccgttaaagagttgcagatagtagatctggactacaaggagaatccacaggcagacttcagctgatatgaggaaaaactctctcgttattagagttgcccaacttttgagtaataaatgcatagccaccagaggctacctgaccatgcccatgggtgaaagctgtggtagcaggggtccctgtgacacaataatagaaagctggacctaatgacctctgggtcttgccactctaaacttccatgactctcatcaatgggttgaaagtacttcattccattaaacctctattaagtgccatttcccctattaatttctaagaaagtaaatctctctgctaaatctaaccactggaaataatcaaattcaccactattctcacagcccagtaggctgctatcttccatcttctttgtcacaatgttgcaagtggcctcagatacttgactttcgccatatgtgtctttccagcctgcttccacttcctagtccatctctcaacaatctcccctccccacctctcattcctccttgcactgacttcatttctcattagaagcaggtgtcagggcgaagagaggaaaacaaggtcaaggaagtgaggcagaatggagtattcagagcccaaattttcttataaagaaaatcactttgaagggggaagataagtgggagacgaaaacaatgagctgacacttatgccatagtctaccttccagggagcaggcagtggtgctgccaccaaggcaccagagtgatgattttcttgtctccagaataatgacttcccacaatggccaaagacaactgaggtcaggtgctctgtcctagcttttataccattgagtgagggggtggggaagggaaaaatataaaaggatagaaaggaaaggaataaatgaagccagggccatttgcgccttggagaaatggctaggtatgagggaggaataagggttaaaactagttagggagattactgggtgttgacagaaaaaataaaagtcagttcctgagaggtgaagaagaatagagcgcctcaatgcagtcactgtcaccttggatgctaaccattccagagggcatctgatgatcaattcaacatcctgctgtttctcttggcaccccaatcaggatcctggagtggctaccacaagactcacctatatcagaggacactgggttaatgtaaaaagctgaaggatactgattagggtagaagtcttacatgtttggaccaaatccaatgtggacaaagtagctgagcagcaggaagttgaggggtccacagctgagcctggtgtactccccagagcattctccagatggctcgaattaccacaatcatgcttcaattaaaactgtcataaaacttgggataggggtttggaagaacagggcattgaaagtgcagagaaaatgtagagtgtatagaggtgactgaagagggtgatagaaagaagtgtccttccaccaaaacatccatttcttttggttggaaggcaaggactggaaaagaggggtgggggcagcaaatgctgtccctttctttcctcataaatctggagcctagcctacttggacagtttgctgatgactctgatgagggcaccattttcatctttcagcctctggttgtcggatttcagttctgttaacaccttcatttcttcctccatttctgacattttgcgctccaaggctcgcctctcccgtttctccatctccagcactgatgatcggtcagaggtcttttcttgtttctgctgggccaccttctcaagcttggactttatatctgctagctctagctgggcttcctgaagttttgttttcagtttttggttttcagtcagagcactctcatagagttttttataatctctgttgctgtcttcttctacacggctggtcagggtggctaggcgggcctcccgggcctcccgacgggctcttgctgaagcccggtcaccgtaagaatcactggttgtaggattactacctcccgattccaacctagaaagtctttcatgctatgtcaaggacagcagaagaatgctgatgctctacccactgaatcttgatactctgagtaggcttttaagttgtccttcaagaagacgttccttcactcaaggaggtgagatgctactagcaagtcaattcgaacatgtaacccacgtttctttgacctcttcagagccatcagtttcatcctcatcctttgtccagaaattgatgcctgtgcctcttcgtcgttccttgggccgcctcctctctcggatggacagcctcttagaggactgctcatccaaatctgcttcttcattctcatttttgtccatttcctttgcagttgtagtgtttgtggtagtctctgaactctcagaatcagggactgaaaatctatttgtccatagcaggtgggaactggtgtagagtgagggtcttgacgtagaaggagatgctggcgtggtgggtttgtctggctgagctgggcacctcaggcgatgacagataggctcttcatccagactcctgccccagggctgctggccctccccagcttctgttgctggaactgctgagggctcatgcttctcagggctcccctcaagcccttcagtgtctgtgggcttctcacgaggctgctcctgagcttgcctctctgccctcgaccggctgaatgtcctttctgcttcttgaaggtctgttagggtgacaccttgagtagaccttcgtgtctgccgagcttgtctggagcgtgctttccgtaaagactctgcttcctcatcccgtacaggagtcagataggacctcctcttctccctggcttccacagaggaatctgttccagtaatggagagcacaggagtagctgtaaccccattggcagtgctaggaagagggcgattggtgatcacacagagcggggtgctagaagagacattgtctgctgttttctctgctgttgtgtcggcctgggatttgtgaggagtccttttcaagtaagttgatacataggtggagggagcaattgtctgtgggatttcatttccttttgcttcatccctccatagctgccgggtataggagccactcctcactagattaacagctgattctctgttctccttttcttcaatatcacttgtgctgttgagcttccggggtgctagtgaactaatatagcttttgttttctctctccttatctttgttgtccagtagagcagaaatccgagggcttgaagaggagcgatagatggaagagcctcggtcccttataggttccctggaattggccacctcactcagcatgttgtggctgccagtttttctcagtcccaatctccatgaagaaggagattcatctttgggctcttctggcttgttaaaaaggccagaagagaacctcctagcagaagaggcagagaaggtattttgagctggtgctggtatctgctctgtgatactactcttgctttcagagttggaatgattgacaaaggcttctggctttttatctgcctccttctcagtttctgactcagaagcttcatcttcaccttcctcctcctctgagctggagctactagattctttattttcttcctccatttcttgggacttaggtgtctcctcctcatagagcatcttctctttgttcttaaagaacccactctgaatcttgctgttcagatctgactcaatgagtttattccgtgtctccttttcacttcgaagcacattctgcttcttctggagcaactccaaatgctccacgagaccctcatcagccacatcaaatggtgtctggcccagtttatttcgaatatccatgtcacaaagtgcttctgccaggatggagcaagcctccttcactccccagtgtgcagcagcatggaggggagtccagccatcataatcctgaacattgagttcatagccagcctgaattaaaagtctgaggacttcagagtagcccttggcagcagccacatgaagggctgtagcccctgagcgagcctgcctcacatcctctattttcccactgttgagccactggcgggcatcctgcaacatctgctgctcttcttcttttcttgactgctctagatcaactccttgcttctttacttgctccagaagaagatccttcatggctggctcttctgcaaggtcagagggaacttcaccttcactattgacaatacctacactggctccgtgattaatgaaatactctgctatgttgagatagccacaggaagctgctgcatgaaggggtgtccagccctcgttgtcttgctggtttacattggctctgttctccaccagaaacttcaccatgtccaaattttcatcaatacatgcctggtgcagggctgtcaagccgtccacgttgaccgtgttgatatcagcacctcttgccagaagctttctcacctcgtcggtgtccccgctagagcaggcggccagaaagacagcaccgtcctcgaagcggaccctggggctcccgcgcctggtcagcggctgccgccccgcgcctcgtcgctccgcaggctcctgctctgtcagcgagccccgccagcgccgaagctgctctgcccgccgcattcgcgccgactctgcccgcttccctcctaggtgctccagttccgccattgctccggcctcggcagctgctgccaaaactaccaacactaaattactgttggggctcgagttgccgctgccgcctctctcagagcgcttcagcccggagcagagggcggagaccctcgcgccgccatctttactcctcccgccagtagt

SEQ ID NO: 15199 - RNA, 2665 nt, Homo sapiens
  source 1..2665: mol_type = other RNA
gctgggattacaggcatgagccactgcacctggtggaattgggatcttgaattacagcttctagtttaaacagcatgtggtgtttcagagggaggaccatggagagctacatgtcatgttaggaaagaattaacagacagaggtagtatatattaagggaatgaaccactctaaacactgaatatcactggcaaccctaaaatgatgaggatttaatgacttgcacactcaagtgaaccaagggataaaactcctacaaaaagaaaatactgtaagtattaatgctaggttatcatcaagaactaatggtttaattttgcactggatttgtattctttccaggcctggacatgatattttaaaggctggttttgtctagaggaggatggccaagatgtgacaggtaagaaaagcatgccatatgaggaatgacttaaaggactagagtaacagcagctcaaagtaagactgagggggagaccacccactgcacatatctcaagtgccgttaaagagttgcagatagtagatctggactacaaggagaatccacaggcagacttcagctgatatgaggaaaaactctctcgttattagagttgcccaacttttgagtaataaatgcatagccaccagaggctacctgaccatgcccatgggtgaaagctgtggtagcaggggtccctgtgacacaataatagaaagctggacctaatgacctctgggtcttgccactctaaacttccatgactctcatcaatgggttgaaagtacttcattccattaaacctctattaagtgccatttcccctattaatttctaagaaagtaaatctctctgctaaatctaaccactggaaataatcaaattcaccactattctcacagcccagtaggctgctatcttccatcttctttgtcacaatgttgcaagtggcctcagatacttgactttcgccatatgtgtctttccagcctgcttccacttcctagtccatctctcaacaatctcccctccccacctctcattcctccttgcactgacttcatttctcattagaagcaggtgtcagggcgaagagaggaaaacaaggtcaaggaagtgaggcagaatggagtattcagagcccaaattttcttataaagaaaatcactttgaagggggaagataagtgggagacgaaaacaatgagctgacacttatgccatagtctaccttccagggagcaggcagtggtgctgccaccaaggcaccagagtgatgattttcttgtctccagaataatgacttcccacaatggccaaagacaactgaggtcaggtgctctgtcctagcttttataccattgagtgagggggtggggaagggaaaaatataaaaggatagaaaggaaaggaataaatgaagccagggccatttgcgccttggagaaatggctaggtatgagggaggaataagggttaaaactagttagggagattactgggtgttgacagaaaaaataaaagtcagttcctgagaggtgaagaagaatagagcgcctcaatgcagtcactgtcaccttggatgctaaccattccagagggcatctgatgatcaattcaacatcctgctgtttctcttggcaccccaatcaggatcctggagtggctaccacaagactcacctatatcagaggacactgggttaatgtaaaaagctgaaggatactgattagggtagaagtcttacatgtttggaccaaatccaatgtggacaaagtagctgagcagcaggaagttgaggggtccacagctgagcctggtgtactccccagagcattctccagatggctcgaattaccacaatcatgcttcaattaaaactgtcataaaacttgggataggggtttggaagaacagggcattgaaagtgcagagaaaatgtagagtgtatagaggtgactgaagagggtgatagaaagaagtgtccttccaccaaaacatccatttcttttggttggaaggcaaggactggaaaagaggggtgggggcagcaaatgctgtccctttctttcctcataaatctggagcctagcctacttggacagtttgctgatgactctgatgagggcaccattttcatctttcagcctctggttgtcggatttcagttctgttaacaccttcatttcttcctccatttctgacattttgcgctccaaggctcgcctctcccgtttctccatctccagcactgatgatcggtcagaggtcttttcttgtttctgctgggccaccttctcaagcttggactttatatctgctagctctagctgggcttcctgaagttttgttttcagtttttggttttcagtcagagcactctcatagagttttttataatctctgttgctgtcttcttctacacggctggtcagggtggctaggcgggcctcccgggcctcccgacgggctcttgctgaagcccggtcaccgtaagaatcactggttgtaggattactacctcccgattccaacctagaaagtctttcatgtcggagcgtcttggcagtcggggagggagatgctgggggagaatcagactgagatttcctattccgagtgaattctttacttcgggtatataaagaggacatggttcctcaggatgcagatagacact

SEQ ID NO: 15200 - RNA, 4362 nt, Homo sapiens
  source 1..4362: mol_type = other RNA
gctgggattacaggcatgagccactgcacctggtggaattgggatcttgaattacagcttctagtttaaacagcatgtggtgtttcagagggaggaccatggagagctacatgtcatgttaggaaagaattaacagacagaggtagtatatattaagggaatgaaccactctaaacactgaatatcactggcaaccctaaaatgatgaggatttaatgacttgcacactcaagtgaaccaagggataaaactcctacaaaaagaaaatactgtaagtattaatgctaggttatcatcaagaactaatggtttaattttgcactggatttgtattctttccaggcctggacatgatattttaaaggctggttttgtctagaggaggatggccaagatgtgacaggtaagaaaagcatgccatatgaggaatgacttaaaggactagagtaacagcagctcaaagtaagactgagggggagaccacccactgcacatatctcaagtgccgttaaagagttgcagatagtagatctggactacaaggagaatccacaggcagacttcagctgatatgaggaaaaactctctcgttattagagttgcccaacttttgagtaataaatgcatagccaccagaggctacctgaccatgcccatgggtgaaagctgtggtagcaggggtccctgtgacacaataatagaaagctggacctaatgacctctgggtcttgccactctaaacttccatgactctcatcaatgggttgaaagtacttcattccattaaacctctattaagtgccatttcccctattaatttctaagaaagtaaatctctctgctaaatctaaccactggaaataatcaaattcaccactattctcacagcccagtaggctgctatcttccatcttctttgtcacaatgttgcaagtggcctcagatacttgactttcgccatatgtgtctttccagcctgcttccacttcctagtccatctctcaacaatctcccctccccacctctcattcctccttgcactgacttcatttctcattagaagcaggtgtcagggcgaagagaggaaaacaaggtcaaggaagtgaggcagaatggagtattcagagcccaaattttcttataaagaaaatcactttgaagggggaagataagtgggagacgaaaacaatgagctgacacttatgccatagtctaccttccagggagcaggcagtggtgctgccaccaaggcaccagagtgatgattttcttgtctccagaataatgacttcccacaatggccaaagacaactgaggtcaggtgctctgtcctagcttttataccattgagtgagggggtggggaagggaaaaatataaaaggatagaaaggaaaggaataaatgaagccagggccatttgcgccttggagaaatggctaggtatgagggaggaataagggttaaaactagttagggagattactgggtgttgacagaaaaaataaaagtcagttcctgagaggtgaagaagaatagagcgcctcaatgcagtcactgtcaccttggatgctaaccattccagagggcatctgatgatcaattcaacatcctgctgtttctcttggcaccccaatcaggatcctggagtggctaccacaagactcacctatatcagaggacactgggttaatgtaaaaagctgaaggatactgattagggtagaagtcttacatgtttggaccaaatccaatgtggacaaagtagctgagcagcaggaagttgaggggtccacagctgagcctggtgtactccccagagcattctccagatggctcgaattaccacaatcatgcttcaattaaaactgtcataaaacttgggataggggtttggaagaacagggcattgaaagtgcagagaaaatgtagagtgtatagaggtgactgaagagggtgatagaaagaagtgtccttccaccaaaacatccatttcttttggttggaaggcaaggactggaaaagaggggtgggggcagcaaatgctgtccctttctttcctcataaatctggagcctagcctacttggacagtttgctgatgactctgatgagggcaccattttcatctttcagcctctggttgtcggatttcagttctgttaacaccttcatttcttcctccatttctgacattttgcgctccaaggctcgcctctcccgtttctccatctccagcactgatgatcggtcagaggtcttttcttgtttctgctgggccaccttctcaagcttggactttatatctgctagctctagctgggcttcctgaagttttgttttcagtttttggttttcagtcagagcactctcatagagttttttataatctctgttgctgtcttcttctacacggctggtcagggtggctaggcgggcctcccgggcctcccgacgggctcttgctgaagcccggtcaccgtaagaatcactggttgtaggattactacctcccgattccaacctagaaagtctttcatgtcggagcgtcttggcagtcggggagggagatgctgggggagaatcagactgagatttcctattccgagtgaattctttacttcgggtatataaagaggacatggttcctcaggatgcagatagacactcaaccactggattcttcacacaaagctgggaaatttccctgtaggttaccctcacagaatctctccttttgagttgatgcaagatgactttggatagaacgtagagggtattgtgctgagcaacaccttttatgcctagattgagtccttgattctcctcaaaggacacttcttattgagccttgctctccaataaaacctgagtctaggttcctgatgacaccagattaaatcccggaggaaagacgaccttggatcctgccggcagcgagtctgggaactactatcactttatccagagggaagaaatacaaatcctgtggaaatcatgctgtctttccttagcttgactccactgggctgtaaggcatttggaactactatgataaaatcaggtcaaacaacttaaaaaacaaaaacgaaaaatgataaataaggaaccaagagtttataagaaggaagcagtctgaggaagtcaagtttccctaagtcctcccagacgaagctgcttttacatataaacactcacagtcatacacacatcttttcccctcccctcttctattttctgacattccaaatccctattcgctcagtgaggaatgctggagaggagccaagggcaaagattcactttcaactcagaattcgggttaccacttgtaggaggaaaagaaagcctgccagcttctaggaataaagggaggctctttgggggcatgctcagaggcaaacctcaccaaccttccagtgtcccctgcctcagagtaggcagcagtctctaaggctgattgctccgaatactatgagaagggggatttttcaacttctagatctcttaagtaacaacgcccagacagaaaaattagtcaaagcaccttcaggcccttaatgttcaattttaatgagatgccattcctgttgcaccgtgaggaagcaaactgaagctctggctcactgcaaagaaagttatctgtccattacagaccttactggctggatctgtaagtataaagcttaccagagtttcctaagatgccacaatcgggaaaatgacaatggaaagtggtataaaggtgagggaaaagaaagaagggtcagaaatgaagagagaaaacagacagtagtgcaattgcaaggctacaggactcagtagtacagggaaaacgaaattaaaaagagaggaatttatttgcatagtgttgaaggattttggatttgacctggaagaaacatctaaaatttaatcttttgcactttgttgttaccactacactaaccaaaatttctaggccaaatgttttctaagccaacgggtttatccccaaagtaacaaccctcttttctctggactcttggaaactctatcctgctttccctttttccacatgaaatttatacttttcacttcaaactttctcaatatgctattcttttctaactgccttgacaacttctttattcctatgattaactttgtgaaattaaatcaagggaagtgatcaactacttggaagttggtctgaggaatataggttgaaaagagttttacaaactcattcttttagattgagaatgaatcagaacccctttattaggggtcctggaaattattccatcttccttaagaagactgataaattctatcataaaccagaatacagtgtgtctcaaaggccaactgttgccaggtgcaa

SEQ ID NO: 15201 - RNA, 5357 nt, Homo sapiens
  source 1..5357: mol_type = other RNA
gctgggattacaggcatgagccactgcacctggtggaattgggatcttgaattacagcttctagtttaaacagcatgtggtgtttcagagggaggaccatggagagctacatgtcatgttaggaaagaattaacagacagaggtagtatatattaagggaatgaaccactctaaacactgaatatcactggcaaccctaaaatgatgaggatttaatgacttgcacactcaagtgaaccaagggataaaactcctacaaaaagaaaatactgtaagtattaatgctaggttatcatcaagaactaatggtttaattttgcactggatttgtattctttccaggcctggacatgatattttaaaggctggttttgtctagaggaggatggccaagatgtgacaggtaagaaaagcatgccatatgaggaatgacttaaaggactagagtaacagcagctcaaagtaagactgagggggagaccacccactgcacatatctcaagtgccgttaaagagttgcagatagtagatctggactacaaggagaatccacaggcagacttcagctgatatgaggaaaaactctctcgttattagagttgcccaacttttgagtaataaatgcatagccaccagaggctacctgaccatgcccatgggtgaaagctgtggtagcaggggtccctgtgacacaataatagaaagctggacctaatgacctctgggtcttgccactctaaacttccatgactctcatcaatgggttgaaagtacttcattccattaaacctctattaagtgccatttcccctattaatttctaagaaagtaaatctctctgctaaatctaaccactggaaataatcaaattcaccactattctcacagcccagtaggctgctatcttccatcttctttgtcacaatgttgcaagtggcctcagatacttgactttcgccatatgtgtctttccagcctgcttccacttcctagtccatctctcaacaatctcccctccccacctctcattcctccttgcactgacttcatttctcattagaagcaggtgtcagggcgaagagaggaaaacaaggtcaaggaagtgaggcagaatggagtattcagagcccaaattttcttataaagaaaatcactttgaagggggaagataagtgggagacgaaaacaatgagctgacacttatgccatagtctaccttccagggagcaggcagtggtgctgccaccaaggcaccagagtgatgattttcttgtctccagaataatgacttcccacaatggccaaagacaactgaggtcaggtgctctgtcctagcttttataccattgagtgagggggtggggaagggaaaaatataaaaggatagaaaggaaaggaataaatgaagccagggccatttgcgccttggagaaatggctaggtatgagggaggaataagggttaaaactagttagggagattactgggtgttgacagaaaaaataaaagtcagttcctgagaggtgaagaagaatagagcgcctcaatgcagtcactgtcaccttggatgctaaccattccagagggcatctgatgatcaattcaacatcctgctgtttctcttggcaccccaatcaggatcctggagtggctaccacaagactcacctatatcagaggacactgggttaatgtaaaaagctgaaggatactgattagggtagaagtcttacatgtttggaccaaatccaatgtggacaaagtagctgagcagcaggaagttgaggggtccacagctgagcctggtgtactccccagagcattctccagatggctcgaattaccacaatcatgcttcaattaaaactgtcataaaacttgggataggggtttggaagaacagggcattgaaagtgcagagaaaatgtagagtgtatagaggtgactgaagagggtgatagaaagaagtgtccttccaccaaaacatccatttcttttggttggaaggcaaggactggaaaagaggggtgggggcagcaaatgctgtccctttctttcctcataaatctggagcctagcctacttggacagtttgctgatgactctgatgagggcaccattttcatctttcagcctctggttgtcggatttcagttctgttaacaccttcatttcttcctccatttctgacattttgcgctccaaggctcgcctctcccgtttctccatctccagcactgatgatcggtcagaggtcttttcttgtttctgggccaccttctcaagcttggactttatatctgctagctctagctgggcttcctgaagttttgttttcagtttttggttttcagtcagagcactctcatagagttttttataatctctgttgctgtcttcttctacacggctggtcagggtggctaggcgggcctcccgggcctcccgacgggctcttgctgaagcccggtcaccgtaagaatcactggttgtaggattactacctcccgattccaacctagaaagtctttcatgccacgtttctttgacctcttcagagccatcagtttcatcctcatcctttgtccagaaattgatgcctgtgcctcttcgtcgttccttgggccgcctcctctctcggatggacagcctcttagaggactgctcatccaaatctgcttcttcattctcatttttgtccatttcctttgcagttgtagtgtttgtggtagtctctgaactctcagaatcagggactgaaaatctatttgtccatagcaggtgggaactggtgtagagtgagggtcttgacgtagaaggagatgctggcgtggtgggtttgtctggctgagctgggcacctcaggcgatgacagataggctcttcatccagactcctgccccagggctgctggccctccccagcttctgttgctggaactgctgagggctcatgcttctcagggctcccctcaagcccttcagtgtctgtgggcttctcacgaggctgctcctgagcttgcctctctgccctcgaccggctgaatgtcctttctgcttcttgaaggtctgttagggtgacaccttgagtagaccttcgtgtctgccgagcttgtctggagcgtgctttccgtaaagactctgcttcctcatcccgtacaggagtcagataggacctcctcttctccctggcttccacagaggaatctgttccagtaatggagagcacaggagtagctgtaaccccattggcagtgctaggaagagggcgattggtgatcacacagagcggggtgctagaagagacattgtctgctgttttctctgctgttgtgtcggcctgggatttgtgaggagtcctgccatgatgtacagatgcagtagtgtttgcactgattggtgcagggcaagaagaggcaggttgccactggctgccccgagaggtagatgaaccaatggtaatgggtgaggtagcaggagatgaattgcgattggctgaaatgtagggacttgtggggtcactacttctaccaaatgaagcacttttcaagtaagttgatacataggtggagggagcaattgtctgtgggatttcatttccttttgcttcatccctccatagctgccgggtataggagccactcctcactagattaacagctgattctctgttctccttttcttcaatatcacttgtgctgttgagcttccggggtgctagtgaactaatatagcttttgttttctctctccttatctttgttgtccagtagagcagaaatccgagggcttgaagaggagcgatagatggaagagcctcggtcccttataggttccctggaattggccacctcactcagcatgttgtggctgccagtttttctcagtcccaatctccatgaagaaggagattcatctttgggctcttctggcttgttaaaaaggccagaagagaacctcctagcagaagaggcagagaaggtattttgagctggtgctggtatctgctctgtgatactactcttgctttcagagttggaatgattgacaaaggcttctggctttttatctgcctccttctcagtttctgactcagaagcttcatcttcaccttcctcctcctctgagctggagctactagattctttattttcttcctccatttcttgggacttaggtgtctcctcctcatagagcatcttctctttgttcttaaagaacccactctgaatcttgctgttcagatctgactcaatgagtttattccgtgtctccttttcacttcgaagcacattctgcttcttctggagcaactccaaatgctccacgagaccctcatcagccacatcaaatggtgtctggcccagtttatttcgaatatccatgtcacaaagtgcttctgccaggatggagcaagcctccttcactccccagtgtgcagcagcatggaggggagtccagccatcataatcctgaacattgagttcatagccagcctgaattaaaagtctgaggacttcagagtagcccttggcagcagccacatgaagggctgtagcccctgagcgagcctgcctcacatcctctattttcccactgttgagccactggcgggcatcctgcaacatctgctgctcttcttcttttcttgactgctctagatcaactccttgcttctttacttgctccagaagaagatccttcatggctggctcttctgcaaggtcagagggaacttcaccttcactattgacaatacctacactggctccgtgattaatgaaatactctgctatgttgagatagccacaggaagctgctgcatgaaggggtgtccagccctcgttgtcttgctggtttacattggctctgttctccaccagaaacttcaccatgtccaaattttcatcaatacatgcctggtgcagggctgtcaagccgtccacgttgaccgtgttgatatcagcacctcttgccagaagctttctcacctcgtcggtgtccccgctagagcaggcggccagaaagacagcaccgtcctcgaagcggaccctggggctcccgcgcctggtcagcggctgccgccccgcgcctcgtcgctccgcaggctcctgctctgtcagcgagccccgccagcgccgaagctgctctgcccgccgcattcgcgccgactctgcccgcttccctcctaggtgctccagttccgccattgctccggcctcggcagctgctgccaaaactaccaacactaaattactgttggggctcgagttgccgctgccgcctctctcagagcgcttcagcccggagcagagggcggagaccctcgcgccgccatctttactcctcccgccagtagt

SEQ ID NO: 15202 - RNA, 5174 nt, Homo sapiens
  source 1..5174: mol_type = other RNA
gctgggattacaggcatgagccactgcacctggtggaattgggatcttgaattacagcttctagtttaaacagcatgtggtgtttcagagggaggaccatggagagctacatgtcatgttaggaaagaattaacagacagaggtagtatatattaagggaatgaaccactctaaacactgaatatcactggcaaccctaaaatgatgaggatttaatgacttgcacactcaagtgaaccaagggataaaactcctacaaaaagaaaatactgtaagtattaatgctaggttatcatcaagaactaatggtttaattttgcactggatttgtattctttccaggcctggacatgatattttaaaggctggttttgtctagaggaggatggccaagatgtgacaggtaagaaaagcatgccatatgaggaatgacttaaaggactagagtaacagcagctcaaagtaagactgagggggagaccacccactgcacatatctcaagtgccgttaaagagttgcagatagtagatctggactacaaggagaatccacaggcagacttcagctgatatgaggaaaaactctctcgttattagagttgcccaacttttgagtaataaatgcatagccaccagaggctacctgaccatgcccatgggtgaaagctgtggtagcaggggtccctgtgacacaataatagaaagctggacctaatgacctctgggtcttgccactctaaacttccatgactctcatcaatgggttgaaagtacttcattccattaaacctctattaagtgccatttcccctattaatttctaagaaagtaaatctctctgctaaatctaaccactggaaataatcaaattcaccactattctcacagcccagtaggctgctatcttccatcttctttgtcacaatgttgcaagtggcctcagatacttgactttcgccatatgtgtctttccagcctgcttccacttcctagtccatctctcaacaatctcccctccccacctctcattcctccttgcactgacttcatttctcattagaagcaggtgtcagggcgaagagaggaaaacaaggtcaaggaagtgaggcagaatggagtattcagagcccaaattttcttataaagaaaatcactttgaagggggaagataagtgggagacgaaaacaatgagctgacacttatgccatagtctaccttccagggagcaggcagtggtgctgccaccaaggcaccagagtgatgattttcttgtctccagaataatgacttcccacaatggccaaagacaactgaggtcaggtgctctgtcctagcttttataccattgagtgagggggtggggaagggaaaaatataaaaggatagaaaggaaaggaataaatgaagccagggccatttgcgccttggagaaatggctaggtatgagggaggaataagggttaaaactagttagggagattactgggtgttgacagaaaaaataaaagtcagttcctgagaggtgaagaagaatagagcgcctcaatgcagtcactgtcaccttggatgctaaccattccagagggcatctgatgatcaattcaacatcctgctgtttctcttggcaccccaatcaggatcctggagtggctaccacaagactcacctatatcagaggacactgggttaatgtaaaaagctgaaggatactgattagggtagaagtcttacatgtttggaccaaatccaatgtggacaaagtagctgagcagcaggaagttgaggggtccacagctgagcctggtgtactccccagagcattctccagatggctcgaattaccacaatcatgcttcaattaaaactgtcataaaacttgggataggggtttggaagaacagggcattgaaagtgcagagaaaatgtagagtgtatagaggtgactgaagagggtgatagaaagaagtgtccttccaccaaaacatccatttcttttggttggaaggcaaggactggaaaagaggggtgggggcagcaaatgctgtccctttctttcctcataaatctggagcctagcctacttggacagtttgctgatgactctgatgagggcaccattttcatctttcagcctctggttgtcggatttcagttctgttaacaccttcatttcttcctccatttctgacattttgcgctccaaggctcgcctctcccgtttctccatctccagcactgatgatcggtcagaggtcttttcttgtttctgggccaccttctcaagcttggactttatatctgctagctctagctgggcttcctgaagttttgttttcagtttttggttttcagtcagagcactctcatagagttttttataatctctgttgctgtcttcttctacacggctggtcagggtggctaggcgggcctcccgggcctcccgacgggctcttgctgaagcccggtcaccgtaagaatcactggttgtaggattactacctcccgattccaacctagaaagtctttcatgccacgtttctttgacctcttcagagccatcagtttcatcctcatcctttgtccagaaattgatgcctgtgcctcttcgtcgttccttgggccgcctcctctctcggatggacagcctcttagaggactgctcatccaaatctgcttcttcattctcatttttgtccatttcctttgcagttgtagtgtttgtggtagtctctgaactctcagaatcagggactgaaaatctatttgtccatagcaggtgggaactggtgtagagtgagggtcttgacgtagaaggagatgctggcgtggtgggtttgtctggctgagctgggcacctcaggcgatgacagataggctcttcatccagactcctgccccagggctgctggccctccccagcttctgttgctggaactgctgagggctcatgcttctcagggctcccctcaagcccttcagtgtctgtgggcttctcacgaggctgctcctgagcttgcctctctgccctcgaccggctgaatgtcctttctgcttcttgaaggtctgttagggtgacaccttgagtagaccttcgtgtctgccgagcttgtctggagcgtgctttccgtaaagactctgcttcctcatcccgtacaggagtcagataggacctcctcttctccctggcttccacagaggaatctgttccagtaatggagagcacaggagtagctgtaaccccattggcagtgctaggaagagggcgattggtgatcacacagagcggggtgctagaagagacattgtctgctgttttctctgctgttgtgtcggcctgggatttgtgaggagtccttttcaagtaagttgatacataggtggagggagcaattgtctgtgggatttcatttccttttgcttcatccctccatagctgccgggtataggagccactcctcactagattaacagctgattctctgttctccttttcttcaatatcacttgtgctgttgagcttccggggtgctagtgaactaatatagcttttgttttctctctccttatctttgttgtccagtagagcagaaatccgagggcttgaagaggagcgatagatggaagagcctcggtcccttataggttccctggaattggccacctcactcagcatgttgtggctgccagtttttctcagtcccaatctccatgaagaaggagattcatctttgggctcttctggcttgttaaaaaggccagaagagaacctcctagcagaagaggcagagaaggtattttgagctggtgctggtatctgctctgtgatactactcttgctttcagagttggaatgattgacaaaggcttctggctttttatctgcctccttctcagtttctgactcagaagcttcatcttcaccttcctcctcctctgagctggagctactagattctttattttcttcctccatttcttgggacttaggtgtctcctcctcatagagcatcttctctttgttcttaaagaacccactctgaatcttgctgttcagatctgactcaatgagtttattccgtgtctccttttcacttcgaagcacattctgcttcttctggagcaactccaaatgctccacgagaccctcatcagccacatcaaatggtgtctggcccagtttatttcgaatatccatgtcacaaagtgcttctgccaggatggagcaagcctccttcactccccagtgtgcagcagcatggaggggagtccagccatcataatcctgaacattgagttcatagccagcctgaattaaaagtctgaggacttcagagtagcccttggcagcagccacatgaagggctgtagcccctgagcgagcctgcctcacatcctctattttcccactgttgagccactggcgggcatcctgcaacatctgctgctcttcttcttttcttgactgctctagatcaactccttgcttctttacttgctccagaagaagatccttcatggctggctcttctgcaaggtcagagggaacttcaccttcactattgacaatacctacactggctccgtgattaatgaaatactctgctatgttgagatagccacaggaagctgctgcatgaaggggtgtccagccctcgttgtcttgctggtttacattggctctgttctccaccagaaacttcaccatgtccaaattttcatcaatacatgcctggtgcagggctgtcaagccgtccacgttgaccgtgttgatatcagcacctcttgccagaagctttctcacctcgtcggtgtccccgctagagcaggcggccagaaagacagcaccgtcctcgaagcggaccctggggctcccgcgcctggtcagcggctgccgccccgcgcctcgtcgctccgcaggctcctgctctgtcagcgagccccgccagcgccgaagctgctctgcccgccgcattcgcgccgactctgcccgcttccctcctaggtgctccagttccgccattgctccggcctcggcagctgctgccaaaactaccaacactaaattactgttggggctcgagttgccgctgccgcctctctcagagcgcttcagcccggagcagagggcggagaccctcgcgccgccatctttactcctcccgccagtagt

SEQ ID NO: 15203 - RNA, 5321 nt, Homo sapiens
  source 1..5321: mol_type = other RNA
gctgggattacaggcatgagccactgcacctggtggaattgggatcttgaattacagcttctagtttaaacagcatgtggtgtttcagagggaggaccatggagagctacatgtcatgttaggaaagaattaacagacagaggtagtatatattaagggaatgaaccactctaaacactgaatatcactggcaaccctaaaatgatgaggatttaatgacttgcacactcaagtgaaccaagggataaaactcctacaaaaagaaaatactgtaagtattaatgctaggttatcatcaagaactaatggtttaattttgcactggatttgtattctttccaggcctggacatgatattttaaaggctggttttgtctagaggaggatggccaagatgtgacaggtaagaaaagcatgccatatgaggaatgacttaaaggactagagtaacagcagctcaaagtaagactgagggggagaccacccactgcacatatctcaagtgccgttaaagagttgcagatagtagatctggactacaaggagaatccacaggcagacttcagctgatatgaggaaaaactctctcgttattagagttgcccaacttttgagtaataaatgcatagccaccagaggctacctgaccatgcccatgggtgaaagctgtggtagcaggggtccctgtgacacaataatagaaagctggacctaatgacctctgggtcttgccactctaaacttccatgactctcatcaatgggttgaaagtacttcattccattaaacctctattaagtgccatttcccctattaatttctaagaaagtaaatctctctgctaaatctaaccactggaaataatcaaattcaccactattctcacagcccagtaggctgctatcttccatcttctttgtcacaatgttgcaagtggcctcagatacttgactttcgccatatgtgtctttccagcctgcttccacttcctagtccatctctcaacaatctcccctccccacctctcattcctccttgcactgacttcatttctcattagaagcaggtgtcagggcgaagagaggaaaacaaggtcaaggaagtgaggcagaatggagtattcagagcccaaattttcttataaagaaaatcactttgaagggggaagataagtgggagacgaaaacaatgagctgacacttatgccatagtctaccttccagggagcaggcagtggtgctgccaccaaggcaccagagtgatgattttcttgtctccagaataatgacttcccacaatggccaaagacaactgaggtcaggtgctctgtcctagcttttataccattgagtgagggggtggggaagggaaaaatataaaaggatagaaaggaaaggaataaatgaagccagggccatttgcgccttggagaaatggctaggtatgagggaggaataagggttaaaactagttagggagattactgggtgttgacagaaaaaataaaagtcagttcctgagaggtgaagaagaatagagcgcctcaatgcagtcactgtcaccttggatgctaaccattccagagggcatctgatgatcaattcaacatcctgctgtttctcttggcaccccaatcaggatcctggagtggctaccacaagactcacctatatcagaggacactgggttaatgtaaaaagctgaaggatactgattagggtagaagtcttacatgtttggaccaaatccaatgtggacaaagtagctgagcagcaggaagttgaggggtccacagctgagcctggtgtactccccagagcattctccagatggctcgaattaccacaatcatgcttcaattaaaactgtcataaaacttgggataggggtttggaagaacagggcattgaaagtgcagagaaaatgtagagtgtatagaggtgactgaagagggtgatagaaagaagtgtccttccaccaaaacatccatttcttttggttggaaggcaaggactggaaaagaggggtgggggcagcaaatgctgtccctttctttcctcataaatctggagcctagcctacttggacagtttgctgatgactctgatgagggcaccattttcatctttcagcctctggttgtcggatttcagttctgttaacaccttcatttcttcctccatttctgacattttgcgctccaaggctcgcctctcccgtttctccatctccagcactgatgatcggtcagaggtcttttcttgtttctgggccaccttctcaagcttggactttatatctgctagctctagctgggcttcctgaagttttgttttcagtttttggttttcagtcagagcactctcatagagttttttataatctctgttgctgtcttcttctacacggctggtcagggtggctaggcgggcctcccgggcctcccgacgggctcttgctgaagcccggtcaccgtaagaatcactggttgtaggattactacctcccgattccaacctagaaagtctttcatgctatgtcaaggacagcagaagaatgctgatgctctacccactgaatcttgatactctgagtaggcttttaagttgtccttcaagaagacgttccttcactcaaggaggtgagatgctactagcaagtcaattcgaacatgtaacctgccacgtttctttgacctcttcagagccatcagtttcatcctcatcctttgtccagaaattgatgcctgtgcctcttcgtcgttccttgggccgcctcctctctcggatggacagcctcttagaggactgctcatccaaatctgcttcttcattctcatttttgtccatttcctttgcagttgtagtgtttgtggtagtctctgaactctcagaatcagggactgaaaatctatttgtccatagcaggtgggaactggtgtagagtgagggtcttgacgtagaaggagatgctggcgtggtgggtttgtctggctgagctgggcacctcaggcgatgacagataggctcttcatccagactcctgccccagggctgctggccctccccagcttctgttgctggaactgctgagggctcatgcttctcagggctcccctcaagcccttcagtgtctgtgggcttctcacgaggctgctcctgagcttgcctctctgccctcgaccggctgaatgtcctttctgcttcttgaaggtctgttagggtgacaccttgagtagaccttcgtgtctgccgagcttgtctggagcgtgctttccgtaaagactctgcttcctcatcccgtacaggagtcagataggacctcctcttctccctggcttccacagaggaatctgttccagtaatggagagcacaggagtagctgtaaccccattggcagtgctaggaagagggcgattggtgatcacacagagcggggtgctagaagagacattgtctgctgttttctctgctgttgtgtcggcctgggatttgtgaggagtccttttcaagtaagttgatacataggtggagggagcaattgtctgtgggatttcatttccttttgcttcatccctccatagctgccgggtataggagccactcctcactagattaacagctgattctctgttctccttttcttcaatatcacttgtgctgttgagcttccggggtgctagtgaactaatatagcttttgttttctctctccttatctttgttgtccagtagagcagaaatccgagggcttgaagaggagcgatagatggaagagcctcggtcccttataggttccctggaattggccacctcactcagcatgttgtggctgccagtttttctcagtcccaatctccatgaagaaggagattcatctttgggctcttctggcttgttaaaaaggccagaagagaacctcctagcagaagaggcagagaaggtattttgagctggtgctggtatctgctctgtgatactactcttgctttcagagttggaatgattgacaaaggcttctggctttttatctgcctccttctcagtttctgactcagaagcttcatcttcaccttcctcctcctctgagctggagctactagattctttattttcttcctccatttcttgggacttaggtgtctcctcctcatagagcatcttctctttgttcttaaagaacccactctgaatcttgctgttcagatctgactcaatgagtttattccgtgtctccttttcacttcgaagcacattctgcttcttctggagcaactccaaatgctccacgagaccctcatcagccacatcaaatggtgtctggcccagtttatttcgaatatccatgtcacaaagtgcttctgccaggatggagcaagcctccttcactccccagtgtgcagcagcatggaggggagtccagccatcataatcctgaacattgagttcatagccagcctgaattaaaagtctgaggacttcagagtagcccttggcagcagccacatgaagggctgtagcccctgagcgagcctgcctcacatcctctattttcccactgttgagccactggcgggcatcctgcaacatctgctgctcttcttcttttcttgactgctctagatcaactccttgcttctttacttgctccagaagaagatccttcatggctggctcttctgcaaggtcagagggaacttcaccttcactattgacaatacctacactggctccgtgattaatgaaatactctgctatgttgagatagccacaggaagctgctgcatgaaggggtgtccagccctcgttgtcttgctggtttacattggctctgttctccaccagaaacttcaccatgtccaaattttcatcaatacatgcctggtgcagggctgtcaagccgtccacgttgaccgtgttgatatcagcacctcttgccagaagctttctcacctcgtcggtgtccccgctagagcaggcggccagaaagacagcaccgtcctcgaagcggaccctggggctcccgcgcctggtcagcggctgccgccccgcgcctcgtcgctccgcaggctcctgctctgtcagcgagccccgccagcgccgaagctgctctgcccgccgcattcgcgccgactctgcccgcttccctcctaggtgctccagttccgccattgctccggcctcggcagctgctgccaaaactaccaacactaaattactgttggggctcgagttgccgctgccgcctctctcagagcgcttcagcccggagcagagggcggagaccctcgcgccgccatctttactcctcccgccagtagt

SEQ ID NO: 15204 - RNA, 14760 nt, Homo sapiens
  source 1..14760: mol_type = other RNA
gctgggattacaggcatgagccactgcacctggttgtattgtgttccttaggacagctaccatgtcattgcactttgctgcctaattcagtaacaattcatactccattgtaccttaaaagcacaatgatatttgaaatccacttttcttgtatatattggtaataaaaaataaaatgttgtagcatgggaatacaagtggcattcaaaatgctgctgagttataactgtgtcactgcaatttacattgcacagagcggcagggcaaaatgatgagaatgccacatattctcatcatacggtctctgcagcaactactcaattctgccacagtagcaccaaagtggccgtggacaacttgcaaatgaatgtggttatgttccaataaaacttcatttatggacactgaaattcaaatgtcatataatttccctatgtcctgaaatatcatttgatgtttttcagccatgtaaaatgtgaaaatcacccttagtttggtgagccatacaaaaacaggagggtaccttgctgatgcctaatctgcaatgggcaggaaacagaagccaaagtcgtccctgctcttccagagctctcctgttcctgaacagccgatagccctggaaggatgtgataacagcagcaggaaagcaggttgatgcttcagggagacaaaaactaaagcttccctcatagtcattagaacataatgaatctctcttattttttcttccatttacaaccctacttccacctttgttcagggtcctggagagcctcccagcttcttttaatcccggggcataatcctggggccccctctcacaaagaaaggggcctaaacgaaaattcatcagctgtgtgcagtggctcctgcccgtaatgggaggctgaggcagaaggatcgcttgagcccaggggttcaagaccagcatgggcaaaaaagtgcgacctcaactctacaaaatataaaataatttagccaggcacagtggcatgcgcctgtggtcccagctacttgggaggctgaggcaggaggatcgcctgagtcccagaggtggaggctgcagtaagcagagatcataccactgcactgcagcctgggcaacacagcaagaccctatccctaaaaaataatactaagaattgatgaagactaatctatgaagactaacatgtgggagaagcaagaggggactgtggaagccacatggggaagcacacactgtggagcgtcacccagcagtgtcccagcaccctggagctgctgctgctgcagacagcctgaaccagcagtggggaaagcggaagcagagcaggaactgtggatcctggaaacaagaaggggagaaaatgaccttgggaacagagaaatgggcaaagagcaggcttttgagaaggaaggaggaagcagcattgcatcactcagacttgattcttcagagcttcctggaagtgattctagtttcacaattaaacgagacgattgtcggagagaaacctgttcaacatctccaaattcatggacggttttgccaaaataaaaattttgtaggcaccagtgtggttcattaggacaatacaggcatccttcactacattttccctagccctaagcctagtgtctacattaattgatattaaattagtctcgcccctaaccctgcttctagtggtcacagcagctacagggaccatccagctgaaggtcttggtatgtgatctcgaaagtcaaggtcagcgtggagaactggaaagaggcctgactagaagacagactgtcgctggtcagttgtgtcatcttctgcaagttgcttaaacctgttaagttttctcactctaaagtgaggtgttggggcagtgtctctgactttgaatgtgcatgaatgacctggggaccttgttcaaatgcagattctcatccagtggtctgggctggggcctgagattttgcattgctagcaagcacccaggtgatgctaatgtcgtcagcccactgactacactgggcagcaaggggctggacaatcttctatcccttgatagatctaaaaaccatcctagggctgaggaagctgcaatgatgttaatttttagaacatacaagattctcttatttacgtatcctaggctgtcctcccaactccctctaggtcatccccttcgccatcagttgcctatatgagaatgaccagaaattggccattcccaggcccgactttcccctcctccatccattctttcagatgcctaccggacatctccacaacgttctcctacaagcccttagcactcaaagtcctcaaactctgggaggaagcctgactcctctcttttcacccctactcccagcatccattcagtccccgaggtctgtcagctctccttcctaaatagctctcgactctgtccacttataaactgatgctggcaagcctcctcaccttcgaatggcctgttgtcttctcctagattctagggcattcccaccaggataacacccattcctccattaggtatcagctagaacttcagttccttgggaatacagcacttcacagcctctctggattagaataaggtctctgttcacactcttttaaaaacactgggcttacttgtaattacttatctttcccacttataacaacaaaatgtgacatgctttttgtcctcatccctaagacctagctaagtgctttgcacatgactggtgttcaattaatatttgttgatttctcttatatagttctcacaccagctgtcccaagaccgtttgctggtaagacattcttcttcttcagggtaggactttttgttcatttttaaattgtttccagggttagtactgattgttttctttgattcagagtgtctctgcagggagtaggggagatatttcaagttcactgttttaattttgccagtaaaaggaaatttaccgttttgcttcttgcatctagtcactgctagccgcccccacttctagtgaagatggtcagaactctaatacgcaaacaaaaccgagctggggagaaagaccacaattagtgaatacgcacgtgggagccctccctggacaagctcctcatctgaattcttcaagactacagaagatgttaagtagctgtcattacataatcagtgggagatgccttcagaaacatccgcctacagaaagaggtagcccgtctctccagcacccacattcctgggcgagggtgacactccagtcagaaggtaagaatcccatgtaagcgctctgtgaagagcaaaccaccactcaattggaatacagtagcagtcctggaggaatccaggactccaagcgcactgagccctgtagatctcacccagcggtgagcgctggagcccctgctgggaggacccatcgtgccaaaggcctctgagcgcagagctgcccagactggccagggacaagacctggagctgctgggaagcacaaaagctcatccaatttacttctcccagaaatatcttatctacctgaagtgaacagttaaatcccatgattaggtcccttgtttcagcttcatcatccatccaaatccacggcccattgtaatgcaaatcatgtatagtctaatgcaaacaaacagacttttatcctaagacatttttgtccttatatttgatacaaggagaggatgatactttaggaataacaggctaatactgagagaacccaggctcgatgtagtcacctaatattatcaacaaagtcaacagaataaagaagaagaaaaaagcagcaattatttccttactgctttcaaaatgtgggttacaacctattacatttcaaaagcttccccgataatatccctgttttatttataaacttaagagctgatttctgtcaccctcatctcttcctatctacatcaaacctctgaaggctaaaaatgtaacagactttccttggagtgggagcaaagggtggggactggcccctggatgcgtgatcacaagggtctaatgaccatgcctgttcaaaaacagacccttaccacagttattcctccaggcagtctccctgaggttgtacagagaaattctactgaaaacccatccttataaaacatttaaatatcatatagtttatcaaggcaaagcaaactaccgaaaaactccctcacacctgtaatcccagcactttgggaggccaaggcagatggatcacaaggtcaggagactgagaccatcctgcctaacatggtgaaaccccatctctactaaaaatacacaaaaaaaattagccgggcgtggtggcgggcgccagtagtcccagctactctggaggctgaggcaggcgaatggcgtgaacccaggaggcggagcttgcagtgagccgagatcgcgccactgcactccagcctgggcgacagagcgagactccgcctcaaaaaaaaaaaaaaaaaaaaaaacttcccacaacaaacctcaaaactcttaaatagatgcagggactgtgcggtatgcaaaaccaactagtaaaggaatgttaacacctagtcccagactccaaaaataaaagtcagctggaaagcaatgctgtttagccctccacggagaacactgtccacctcatttccctgcattgtttgctgtatttacgtagaaaaagaagttccattcaggctgtggactccgctgtttagccgcatattatatttatcggacactttctacatactaggcattgtgctttctgcggacattacctcactgaggcatgcacagcatctcctaagtggacactataggtatctccattgtacaaagcggacagtaatccttgcgcaagttgagcagcgtacccagggtcacgaagccaatgagaggagcagtgggatctgaacctctttgggattctagagagggaaactgtaactactatacagagctggtggctggtgccctgggaaacccttcaccggcttacaagaccagatgagactgagatataaaggaactaattccattcccactgttgggaaataacatgtgccattctcatgggacatctgagagctattaatgaataggatgttacactgacccatctccacaagggaagacaacaaaaaggaacaaactgtgtaagttttatatacttacatctggcaatttctgcctttcccggaggcttgtttataacattttgtaatgcaccataaattgaaaattttaattatccattactctatgtaaactttggtaatcaaactccatttcaagatgttcttggggctgggtgaagtagctcacgcctgtaatcccagcactttgggaggccgaggcaggtggatagcttgaagtcgggagttcaagaccagcctggccaacattgcgaaaccccctctctatcaaaaatactattagctgggtgtggtggtgtgcacctgtaatcccagctacttgaaaggctgaggcacgagaatcgcttgaatctgggaaatggaggttgcagtgagccgagatcacacccctgcacaccaacctgggagacaaagcaagactgtctccaaaaaaaaaaaaaaaaaaagtccttggattcagacttccgtcatattagccacacgcctcttcttgccagagtcctgcctggctgcaggttcagaatggcccgcaaagtttcagaaaacagagctccaggccccaccccaactctgaatctaaaatcctgctagtgtgatggtcatccgtggttttataaagttctacagatgagtttagtgtgcagcaaggctggacagtcattttaaattgatgagtaccgattgagcagtttgcgatcactagagttcattagtcatttctttcctggatttgcgggcaatggaagtgggagtggtgcctgaagtgagctcctccccacctcgtggcatcacctcttcagcagaacaaggcttgtctgtgatgtacataaaaacgctctttctcatgctatttcactgcattccgcttttccgctttaaatctttacagacgtgagccaccacgcccagcctatttatgtttgagaggcccaggctggaggatcacttgaggccagcagtttgaggagcgcctgagcaactcagcaaaaccccgtattaaaaacagccaggcatggtggtgtgcacaggtagtcccagctacttgggaggctgagatgggaggatcacctagcccagttgtttaaggctgcagtgagctgcaatcacaccaccaaactccagcttgcgtgacaaagccagacaccgtctctaaaattaaagaagtaacattaaaaaaaacttagccgtttcatgccactagaggtattttctttcatttcagagggagttaacaaaccccaccccagcagtgcccttctctgcagtctttctgtccaacagtgagtggatgatgattccaaattcatcctcccagggtctcttttaagcaactcaacactttctgctggccacactcaggctcaggcccgtcctcttgcctgggtgttcattaacaactccctgcccggcacacctgcttggctgcttcctggccaccctagtgcagaactaccacacacacccagtgcctgccactttattttgcccttggctctgaatctcccgtgactgcagtttcagatatggaattcaggggcaagtacactgactaatgaatgagtatataatggaagcaaaactttacaagaataaagaaaaaaattcccaaagtagcaattttagaaatttaatcgggaagattatcaaatagctggtctttcagacagatgaaacattaagcacttatacctacacggcctttctctagctatgagaactcggccaaccacacccatgccagcatcgcccggcctcccatgcgaacagagctgggctccacttgtcttgtccacttgtttcctctgtcctgcatcatgaacttttgccaccactttgcctgacccaaacttaatgcactttattaatagtcaacatgactcaggctctagtactgtgctccttcaggacccagctgggactgaaccaggctacctggtaaaagcgaagggaagccggtttaagacttgtctctgcctcctctatgctttgaagaaggattcacaggttttgctggggatgacaggaaattcaactgaaatggaaatttacccacattaattccacacctgataacagggacataccctaaagatgggaaattatggggaaaaattttcaggtacagcagctgcatactggaagagagacctgtagcattctagttgtgtttcaaatcagcgtccagttggagaaacactttgtctcctaagatttaaagtaggaaattagaaataaatactgacaaatacctgacagtctcagtgttaaggtagtgttattttttttaaagttctgatgcaagaacacccactgagagcagccaaaatctgggaccttggctatgcataatgccaaagagagccaaacacaccaagcgatgagccacttacctcaatgaacatgtcttccacaaaacaagcatccagtgccttcaacacaggcatacgtcaaaaattcctggtccagggtgaaagcccagtaggcatccacaggctggttctcagtggattcatttggattaaggttagtcattaaaagggaggataacaaataagctatcttcttagggtttcttctcttgttctttgtactacaaattacttggtgatgtatgttttcacgcaaggaaacaggcctagataagaaaccagggttatgaaaatcagaacttctcctctactctccctgacaccaaaggttttccaacgtctggtcaacagacatccctagcagatttttaagaaatctgaatgaagtctgggtataccgaagtcacgcacggcttttgtccccattacattttcaaacttccttcatatatagcagtaagaccaagtcatgtatttggaatgaaccatctggtctattacatacagtctaccactataaaaatggacataaaaatgagtcttgaacttgtattctgtctatggggataccacccagaatgcaccggatcgcatctgaacctgcattctgcgactatcaaaataaaggcaggcccaaaggaaactgagaaactggcctagaactgagtgcctgctatctcgtcttcgtgtgtattttgattatgtatctccctattggaagaacagaaaagttcaacaccacaaaagctgggaagcagtacaggggcaaactcaatggtcacttgtgagcctaacataattactgaatctttcatgattttttacatgtagttttaaataaaaatgtcggtttttttttttcagcccaatatccatgtgcctaggtaaaattctcacaccctaagaagaaaactaatggaagttttcctttcttacatgtggttaacttcaactttacgcaaccaaccttaattttacagattcacgcttaacttttaaataagcatcttgcctctcgaaagccaccttaatatatactgaagcaggtgaatttgtaaaaagagaagactttaggttagcaattgaatcacagtggcaagaattctagaattctgatatggccccgtacgaggagttagggaaggaagaatgagtattcgtattccttccttcatccaagcacgtcaaagcatatcagagaaaaccatcagaccctcacatccagtcgaaatgctaccaactaaaatatgagcattttgaatcacaaaattatgtaaacattcaaataaaaaaatcaatgtgaaaaatcaaaatgatctgttaaacctccaatttttactttcagagattgctgatgcctatgtcaatgtatctcaaatagtttcctttttacacatttaactcaactttgatactatacctaccagacctggaccagtttaattgcataggaagatttttactatgtttacatttttcttaaattaatttttaaaaaagcatagtaaagagtctgaggacaaattattcaactgtttatcatacataagaccgcatgactataatacaaaggggggttcttttttcatttaacgttacaatatacacagcaagtccggactagatcttacaatctgaacacaggtatttaaccttttccatgctgtttatgtttacaatgcacagaagtcctgtaaccaaactgtgtagtaaagcacacaaaactggactgtaacataacacagtatgcagaagcattggattttatgattttctttacgtaaatatcggtttaaaaactgctttagttttttggtgcttgctaagatgtggcaaccagcacagaaaaaaaaaatgacctgacccatatgatatcttaaccttatattcctaaacagcagtaactactgaattccttttgatattgctatactcaagatgatatccttttattcactgtaaacctttatgaactaccaagttcaaaaaaatcatccacaggcttgacagttaattacaaaataaatatggatttcctgataaacaacaaaaagtttttgtagtttataaaaacgagtatttccaagtttccattcacatttacatagtgtttagcctttcttttctcactgtttacatataaaaacctgcttttgttcagaaaaaaaattgacctagtcagccacatggaattgaccaatagaatgaaacgcggtgttctgctgagtcatcttaaacaggttatcggcagaggtagattactgcttcttttctaggcttcttttgatcctggacaggtaaattacttatcttcattctcccaattcaaccgctcaaaagtgtcacaccccaaaattggtcaatttaaaatgggaacacaaatttagcaactgccagactgtgttacattaaggcagcgtaatctcaacacgaggcacctgttaaataccagcctgtctgctcaggtcacgcatgagagttctgctttgcttgcactcatactctggacctgttggtgcaatcaaggtcttgctttcaagtttacaagtaggttaatcaggaatacaagaatcaactgctggttccatagcttctggatccagtgtccctttaccttcagaagcctgaacacacttagaatgtaacagatgttgtaatcttgaattagatgtcaatctactatgttcagtacacagattgctgtaaatgtattggctatggattcaacaacagttccagttttgtttaagcaatagtacagccataattttcaactgacatttaaaaatggtctagttacaccttgtgtcaaagtgcagaactgctacattattggttacagacatctatgtgctataaaaacagctttggtacaataaattatcaaaaaagaaaataaatttttgtaaaattcacagcataattgtgaggcaaaaaagcagtcacataaaattctgcattttttaaaaatgttcaggatgaacagaagacatctttgtgcagaagaaatggtggagataccacgtgccgagaaaaagcaaaagaaaaagtaaaaagcaggaagggacacagctgtagctatttccatcaaagcaaaccactacttctgtgaccttcaaccaataaggaagtcaactttatgacacacgcaaagtgaccttgcaataccttacaattagtgggtcacaaaagtctattttaaaagaaaggcctcttgaattacccattctctgtgttttcagcattaaggactgtctgcaaaagcatgtccaaaagtgattgcatctgaaatggtaggctcttctaatttcgagtccaaatccataaggccaaaggttatcccaaagaccaccactcagacctccccaggactggccacgaccgacccgttgattgcttctcagtgcaccttggttaggagaccagtcacgttccatcctatcttcctgtggcctctgcaacgggagagccacaggatcccatgtaattgctgctttgctcctcagtaggttcagataggagagttctgatccccgccactcagcatgcttactgtgcctgacaaacttcaccacaaccgtccctttcatacagctgaagatggtgtttgtggaagctggaggtccctcttccttacagtactgcatttccgtgcccaagtgtgtttagaggacttaaaaacccaaatttcccaccctcccacccaaaacaaaacagaacaaaacaaaaaaaaagggggatgggggggacaaaaagaaaaaaaaaaaacaccctcatggggccctttatgcaaattatgtgcagtgccttttactttaaaattagttggcaaatgaccaagaccaacatctgaatattaacttttgctgaatagaaagacaaaaaaaccccactgtgactgggatgtggcaagttaaaatgggggagcaaaaagaggatacctctgagctatccatgaagatgggtttggacatggctcttttaaacacttcaatgtccctttgcaatcttttcaagttaaaaaaaaaatcagctttgccctcttgtagcggttcagtgtgttaatctcctcctgattcaagcagctttgcactttgtttttggaaaaaaaacaccacttctataaaaacacacaagaaacaaactcaagtttcaatgtagtcacgagctagctacaggactctgttgcacacaaactcctgtcatgggggactcttctctatcagccccttgcctcattgtcagatgtccttcagtcatgtaatgtgcaggacctgtattagcagaaaattggtatgttggatgtccagctatgccagtctcttggcggggattggagtagacggtcaaattaacgtccatagctccattctgtccaaagtccaaggtattagcagccactgggcgattctggtaggcctgattgccttggttaccagtagaggaggaagatgtcgaggaagaagtcgttgaggaagacagggatgtcatggagtggtgactgtggccaacctccatagaatcttgggtagaggagctattcgttggagaattgtagacccttggcctggtccggttacccaaggcttgttgtccatggtggtggtgatggtggtggtggtggtgatggtgatgggaactgttaccatggtgatgatgcaatgcattctgttgaggggctacatgaaaggttgtttcttgaacaggatgagtttcaacagtgacctgtgtaggagcttcagtgcctgaccaaccaagaggagcaggaaattgctgacgcacctggggactgtgtgtctcgcagtccatggcctgcacggcagctgtgaagtgcccaccactgtgccgatgctggtgcgtcggatccgaccgggctctcccactgttgcttgtccccgatgagccacctgagcttgacgatgtactggaggtggtgcccgaagactgagactgctccatggcggggcttgtagatacactattacttgtatttgtaccttcatcagctgttttcttgaagaaactgtgctgcagagcataataaggttgaattcgagttttggggtcataatcaagcatccttaaaatgaggtctttgaacttcaagtagtcagcgaccgtatgacctgactccccagcacgtcgcccaccaggtcctcctgtttccactccaagaatgttatgaagtttacgggttcctggtggtttgtactcccgttttccatctttggtcttctttaagttccaagtgccatctggcaacttctcaaagaactttcttgcttttggtgcttggtcaagaatatgagcaggtggaatacccagaacttccactattttattcatctgatctacctcattggcaccactgaacagaggttctccagtgtgcatttcaaccaaaatacacccgagggaccacatatcaatggcaaggtcataaggcattcccagtagcacctctggagaccgataaaagcgactctgaatatactggtatatcctctgccccaactgacaagaactgccaaagtcaactatcttgattgcactgcgtttggggttacaaagaaggatattttcaggttttagatcacagtgaatgatactaagttctggagtcgcaaggaaaagcagtgcagtgcacatctgttgcgcaaactttcgtgttaggttcaaagagacccctcggaaattggtgtttctcagcaagtcatagaggttgtaggacagcatttcaaaaactaaacagagatggtttcgaaacataaagtggcgtttcaaatgcactatgtagtatttcatttcagtgtcatgtttgttcatgagctcaagaagtcgcacttctatctgtgcttgattcagaaaagccttcttgttctttattattttaatggcaacccattcttgctccacacgatcatatgcctttacaacctgtccaaaggaacctttgcctatcaaggagtcaatttcgtaacgatccatccacttttctccgttttttacaatataatcatagttatcatcatcataaccatcattgtaaaccttccgttccttcttatgactagaatcgtctccctggccctgttggtgtcttcgcttcttttttgcatagtaaacctcattaatatgcttgtatgttttgatcaagtcaacagaaagttttctcaggggagcagttgctgggtcacggaaggtttggggcatccgcctctggttagttagaggttgctgaatctggtcagaatatgataaggcagaaacctgttggtcacttatgtttggctggcgacggtcactgtactgatgtgaatggggcatctgtccagccatctgaaggccagcagcatggaatgaaaatgacggtgcaagccgaacagatgaaggtttgcatgctgaagtctctcctccgggacgatggcggggcgctcgcgccgcttcctccggtgagtctcagcctcgggctcccgcgccgcgctcccgccgcggcctccgcagccagcgccgccccggcagcctctctccgcccccggcgctccggctcctggccgcgccgcagcctgctcagtctctcctcggctcgcggttccagcggcgcccggggccggggaggcgacagccccctccccggcaaataccgcagtccccgggccccgattccaggcggcggggccgcacggccggcccggcgcagagggcggcgtcggcgaggccgggcgccgagcggcggctgctgccggcggcttcttcccgaggaggattttgtaaatctcacaaaatggcgcgcgctccgaacctgcgcagcgagaagcgccggggcccgggcggcggcggcggctcctccgccaggagagcccgaaccgcccgcccccgagtccccgcacagacagacagacactcgcacacacccgcacactcgcgcgcacaatcgccctcgcacacgctccctcgcacacacactcgcactcacaccggtcccgcctgctcgccggcggcggcagcggcaccaacagcagcagcaggaacagcagcagcagaagcggcggcggcggcgcccgcaccccccgctcggggtgtccgctctctgaggccgacctgggccgcgatcagcagcagcgacagcagcagtctccccggatacccccgccgcggttgccgccgccacccccgcctcactccaatggggctttttattattattcgggcgggaagcgaaagggtttaaaaaaaaaccaaccaacaaaatggcgacggaccgacccggtc

SEQ ID NO: 15205 - RNA, 14103 nt, Homo sapiens
  source 1..14103: mol_type = other RNA
gctgggattacaggcatgagccactgcacctggttgtattgtgttccttaggacagctaccatgtcattgcactttgctgcctaattcagtaacaattcatactccattgtaccttaaaagcacaatgatatttgaaatccacttttcttgtatatattggtaataaaaaataaaatgttgtagcatgggaatacaagtggcattcaaaatgctgctgagttataactgtgtcactgcaatttacattgcacagagcggcagggcaaaatgatgagaatgccacatattctcatcatacggtctctgcagcaactactcaattctgccacagtagcaccaaagtggccgtggacaacttgcaaatgaatgtggttatgttccaataaaacttcatttatggacactgaaattcaaatgtcatataatttccctatgtcctgaaatatcatttgatgtttttcagccatgtaaaatgtgaaaatcacccttagtttggtgagccatacaaaaacaggagggtaccttgctgatgcctaatctgcaatgggcaggaaacagaagccaaagtcgtccctgctcttccagagctctcctgttcctgaacagccgatagccctggaaggatgtgataacagcagcaggaaagcaggttgatgcttcagggagacaaaaactaaagcttccctcatagtcattagaacataatgaatctctcttattttttcttccatttacaaccctacttccacctttgttcagggtcctggagagcctcccagcttcttttaatcccggggcataatcctggggccccctctcacaaagaaaggggcctaaacgaaaattcatcagctgtgtgcagtggctcctgcccgtaatgggaggctgaggcagaaggatcgcttgagcccaggggttcaagaccagcatgggcaaaaaagtgcgacctcaactctacaaaatataaaataatttagccaggcacagtggcatgcgcctgtggtcccagctacttgggaggctgaggcaggaggatcgcctgagtcccagaggtggaggctgcagtaagcagagatcataccactgcactgcagcctgggcaacacagcaagaccctatccctaaaaaataatactaagaattgatgaagactaatctatgaagactaacatgtgggagaagcaagaggggactgtggaagccacatggggaagcacacactgtggagcgtcacccagcagtgtcccagcaccctggagctgctgctgctgcagacagcctgaaccagcagtggggaaagcggaagcagagcaggaactgtggatcctggaaacaagaaggggagaaaatgaccttgggaacagagaaatgggcaaagagcaggcttttgagaaggaaggaggaagcagcattgcatcactcagacttgattcttcagagcttcctggaagtgattctagtttcacaattaaacgagacgattgtcggagagaaacctgttcaacatctccaaattcatggacggttttgccaaaataaaaattttgtaggcaccagtgtggttcattaggacaatacaggcatccttcactacattttccctagccctaagcctagtgtctacattaattgatattaaattagtctcgcccctaaccctgcttctagtggtcacagcagctacagggaccatccagctgaaggtcttggtatgtgatctcgaaagtcaaggtcagcgtggagaactggaaagaggcctgactagaagacagactgtcgctggtcagttgtgtcatcttctgcaagttgcttaaacctgttaagttttctcactctaaagtgaggtgttggggcagtgtctctgactttgaatgtgcatgaatgacctggggaccttgttcaaatgcagattctcatccagtggtctgggctggggcctgagattttgcattgctagcaagcacccaggtgatgctaatgtcgtcagcccactgactacactgggcagcaaggggctggacaatcttctatcccttgatagatctaaaaaccatcctagggctgaggaagctgcaatgatgttaatttttagaacatacaagattctcttatttacgtatcctaggctgtcctcccaactccctctaggtcatccccttcgccatcagttgcctatatgagaatgaccagaaattggccattcccaggcccgactttcccctcctccatccattctttcagatgcctaccggacatctccacaacgttctcctacaagcccttagcactcaaagtcctcaaactctgggaggaagcctgactcctctcttttcacccctactcccagcatccattcagtccccgaggtctgtcagctctccttcctaaatagctctcgactctgtccacttataaactgatgctggcaagcctcctcaccttcgaatggcctgttgtcttctcctagattctagggcattcccaccaggataacacccattcctccattaggtatcagctagaacttcagttccttgggaatacagcacttcacagcctctctggattagaataaggtctctgttcacactcttttaaaaacactgggcttacttgtaattacttatctttcccacttataacaacaaaatgtgacatgctttttgtcctcatccctaagacctagctaagtgctttgcacatgactggtgttcaattaatatttgttgatttctcttatatagttctcacaccagctgtcccaagaccgtttgctggtaagacattcttcttcttcagggtaggactttttgttcatttttaaattgtttccagggttagtactgattgttttctttgattcagagtgtctctgcagggagtaggggagatatttcaagttcactgttttaattttgccagtaaaaggaaatttaccgttttgcttcttgcatctagtcactgctagccgcccccacttctagtgaagatggtcagaactctaatacgcaaacaaaaccgagctggggagaaagaccacaattagtgaatacgcacgtgggagccctccctggacaagctcctcatctgaattcttcaagactacagaagatgttaagtagctgtcattacataatcagtgggagatgccttcagaaacatccgcctacagaaagaggtagcccgtctctccagcacccacattcctgggcgagggtgacactccagtcagaaggtaagaatcccatgtaagcgctctgtgaagagcaaaccaccactcaattggaatacagtagcagtcctggaggaatccaggactccaagcgcactgagccctgtagatctcacccagcggtgagcgctggagcccctgctgggaggacccatcgtgccaaaggcctctgagcgcagagctgcccagactggccagggacaagacctggagctgctgggaagcacaaaagctcatccaatttacttctcccagaaatatcttatctacctgaagtgaacagttaaatcccatgattaggtcccttgtttcagcttcatcatccatccaaatccacggcccattgtaatgcaaatcatgtatagtctaatgcaaacaaacagacttttatcctaagacatttttgtccttatatttgatacaaggagaggatgatactttaggaataacaggctaatactgagagaacccaggctcgatgtagtcacctaatattatcaacaaagtcaacagaataaagaagaagaaaaaagcagcaattatttccttactgctttcaaaatgtgggttacaacctattacatttcaaaagcttccccgataatatccctgttttatttataaacttaagagctgatttctgtcaccctcatctcttcctatctacatcaaacctctgaaggctaaaaatgtaacagactttccttggagtgggagcaaagggtggggactggcccctggatgcgtgatcacaagggtctaatgaccatgcctgttcaaaaacagacccttaccacagttattcctccaggcagtctccctgaggttgtacagagaaattctactgaaaacccatccttataaaacatttaaatatcatatagtttatcaaggcaaagcaaactaccgaaaaactccctcacacctgtaatcccagcactttgggaggccaaggcagatggatcacaaggtcaggagactgagaccatcctgcctaacatggtgaaaccccatctctactaaaaatacacaaaaaaaattagccgggcgtggtggcgggcgccagtagtcccagctactctggaggctgaggcaggcgaatggcgtgaacccaggaggcggagcttgcagtgagccgagatcgcgccactgcactccagcctgggcgacagagcgagactccgcctcaaaaaaaaaaaaaaaaaaaaaaacttcccacaacaaacctcaaaactcttaaatagatgcagggactgtgcggtatgcaaaaccaactagtaaaggaatgttaacacctagtcccagactccaaaaataaaagtcagctggaaagcaatgctgtttagccctccacggagaacactgtccacctcatttccctgcattgtttgctgtatttacgtagaaaaagaagttccattcaggctgtggactccgctgtttagccgcatattatatttatcggacactttctacatactaggcattgtgctttctgcggacattacctcactgaggcatgcacagcatctcctaagtggacactataggtatctccattgtacaaagcggacagtaatccttgcgcaagttgagcagcgtacccagggtcacgaagccaatgagaggagcagtgggatctgaacctctttgggattctagagagggaaactgtaactactatacagagctggtggctggtgccctgggaaacccttcaccggcttacaagaccagatgagactgagatataaaggaactaattccattcccactgttgggaaataacatgtgccattctcatgggacatctgagagctattaatgaataggatgttacactgacccatctccacaagggaagacaacaaaaaggaacaaactgtgtaagttttatatacttacatctggcaatttctgcctttcccggaggcttgtttataacattttgtaatgcaccataaattgaaaattttaattatccattactctatgtaaactttggtaatcaaactccatttcaagatgttcttggggctgggtgaagtagctcacgcctgtaatcccagcactttgggaggccgaggcaggtggatagcttgaagtcgggagttcaagaccagcctggccaacattgcgaaaccccctctctatcaaaaatactattagctgggtgtggtggtgtgcacctgtaatcccagctacttgaaaggctgaggcacgagaatcgcttgaatctgggaaatggaggttgcagtgagccgagatcacacccctgcacaccaacctgggagacaaagcaagactgtctccaaaaaaaaaaaaaaaaaaagtccttggattcagacttccgtcatattagccacacgcctcttcttgccagagtcctgcctggctgcaggttcagaatggcccgcaaagtttcagaaaacagagctccaggccccaccccaactctgaatctaaaatcctgctagtgtgatggtcatccgtggttttataaagttctacagatgagtttagtgtgcagcaaggctggacagtcattttaaattgatgagtaccgattgagcagtttgcgatcactagagttcattagtcatttctttcctggatttgcgggcaatggaagtgggagtggtgcctgaagtgagctcctccccacctcgtggcatcacctcttcagcagaacaaggcttgtctgtgatgtacataaaaacgctctttctcatgctatttcactgcattccgcttttccgctttaaatctttacagacgtgagccaccacgcccagcctatttatgtttgagaggcccaggctggaggatcacttgaggccagcagtttgaggagcgcctgagcaactcagcaaaaccccgtattaaaaacagccaggcatggtggtgtgcacaggtagtcccagctacttgggaggctgagatgggaggatcacctagcccagttgtttaaggctgcagtgagctgcaatcacaccaccaaactccagcttgcgtgacaaagccagacaccgtctctaaaattaaagaagtaacattaaaaaaaacttagccgtttcatgccactagaggtattttctttcatttcagagggagttaacaaaccccaccccagcagtgcccttctctgcagtctttctgtccaacagtgagtggatgatgattccaaattcatcctcccagggtctcttttaagcaactcaacactttctgctggccacactcaggctcaggcccgtcctcttgcctgggtgttcattaacaactccctgcccggcacacctgcttggctgcttcctggccaccctagtgcagaactaccacacacacccagtgcctgccactttattttgcccttggctctgaatctcccgtgactgcagtttcagatatggaattcaggggcaagtacactgactaatgaatgagtatataatggaagcaaaactttacaagaataaagaaaaaaattcccaaagtagcaattttagaaatttaatcgggaagattatcaaatagctggtctttcagacagatgaaacattaagcacttatacctacacggcctttctctagctatgagaactcggccaaccacacccatgccagcatcgcccggcctcccatgcgaacagagctgggctccacttgtcttgtccacttgtttcctctgtcctgcatcatgaacttttgccaccactttgcctgacccaaacttaatgcactttattaatagtcaacatgactcaggctctagtactgtgctccttcaggacccagctgggactgaaccaggctacctggtaaaagcgaagggaagccggtttaagacttgtctctgcctcctctatgctttgaagaaggattcacaggttttgctggggatgacaggaaattcaactgaaatggaaatttacccacattaattccacacctgataacagggacataccctaaagatgggaaattatggggaaaaattttcaggtacagcagctgcatactggaagagagacctgtagcattctagttgtgtttcaaatcagcgtccagttggagaaacactttgtctcctaagatttaaagtaggaaattagaaataaatactgacaaatacctgacagtctcagtgttaaggtagtgttattttttttaaagttctgatgcaagaacacccactgagagcagccaaaatctgggaccttggctatgcataatgccaaagagagccaaacacaccaagcgatgagccacttacctcaatgaacatgtcttccacaaaacaagcatccagtgccttcaacacaggcatacgtcaaaaattcctggtccagggtgaaagcccagtaggcatccacaggctggttctcagtggattcatttggattaaggttagtcattaaaagggaggataacaaataagctatcttcttagggtttcttctcttgttctttgtactacaaattacttggtgatgtatgttttcacgcaaggaaacaggcctagataagaaaccagggttatgaaaatcagaacttctcctctactctccctgacaccaaaggttttccaacgtctggtcaacagacatccctagcagatttttaagaaatctgaatgaagtctgggtataccgaagtcacgcacggcttttgtccccattacattttcaaacttccttcatatatagcagtaagaccaagtcatgtatttggaatgaaccatctggtctattacatacagtctaccactataaaaatggacataaaaatgagtcttgaacttgtattctgtctatggggataccacccagaatgcaccggatcgcatctgaacctgcattctgcgactatcaaaataaaggcaggcccaaaggaaactgagaaactggcctagaactgagtgcctgctatctcgtcttcgtgtgtattttgattatgtatctccctattggaagaacagaaaagttcaacaccacaaaagctgggaagcagtacaggggcaaactcaatggtcacttgtgagcctaacataattactgaatctttcatgattttttacatgtagttttaaataaaaatgtcggtttttttttttcagcccaatatccatgtgcctaggtaaaattctcacaccctaagaagaaaactaatggaagttttcctttcttacatgtggttaacttcaactttacgcaaccaaccttaattttacagattcacgcttaacttttaaataagcatcttgcctctcgaaagccaccttaatatatactgaagcaggtgaatttgtaaaaagagaagactttaggttagcaattgaatcacagtggcaagaattctagaattctgatatggccccgtacgaggagttagggaaggaagaatgagtattcgtattccttccttcatccaagcacgtcaaagcatatcagagaaaaccatcagaccctcacatccagtcgaaatgctaccaactaaaatatgagcattttgaatcacaaaattatgtaaacattcaaataaaaaaatcaatgtgaaaaatcaaaatgatctgttaaacctccaatttttactttcagagattgctgatgcctatgtcaatgtatctcaaatagtttcctttttacacatttaactcaactttgatactatacctaccagacctggaccagtttaattgcataggaagatttttactatgtttacatttttcttaaattaatttttaaaaaagcatagtaaagagtctgaggacaaattattcaactgtttatcatacataagaccgcatgactataatacaaaggggggttcttttttcatttaacgttacaatatacacagcaagtccggactagatcttacaatctgaacacaggtatttaaccttttccatgctgtttatgtttacaatgcacagaagtcctgtaaccaaactgtgtagtaaagcacacaaaactggactgtaacataacacagtatgcagaagcattggattttatgattttctttacgtaaatatcggtttaaaaactgctttagttttttggtgcttgctaagatgtggcaaccagcacagaaaaaaaaaatgacctgacccatatgatatcttaaccttatattcctaaacagcagtaactactgaattccttttgatattgctatactcaagatgatatccttttattcactgtaaacctttatgaactaccaagttcaaaaaaatcatccacaggcttgacagttaattacaaaataaatatggatttcctgataaacaacaaaaagtttttgtagtttataaaaacgagtatttccaagtttccattcacatttacatagtgtttagcctttcttttctcactgtttacatataaaaacctgcttttgttcagaaaaaaaattgacctagtcagccacatggaattgaccaatagaatgaaacgcggtgttctgctgagtcatcttaaacaggttatcggcagaggtagattactgcttcttttctaggcttcttttgatcctggacaggtaaattacttatcttcattctcccaattcaaccgctcaaaagtgtcacaccccaaaattggtcaatttaaaatgggaacacaaatttagcaactgccagactgtgttacattaaggcagcgtaatctcaacacgaggcacctgttaaataccagcctgtctgctcaggtcacgcatgagagttctgctttgcttgcactcatactctggacctgttggtgcaatcaaggtcttgctttcaagtttacaagtaggttaatcaggaatacaagaatcaactgctggttccatagcttctggatccagtgtccctttaccttcagaagcctgaacacacttagaatgtaacagatgttgtaatcttgaattagatgtcaatctactatgttcagtacacagattgctgtaaatgtattggctatggattcaacaacagttccagttttgtttaagcaatagtacagccataattttcaactgacatttaaaaatggtctagttacaccttgtgtcaaagtgcagaactgctacattattggttacagacatctatgtgctataaaaacagctttggtacaataaattatcaaaaaagaaaataaatttttgtaaaattcacagcataattgtgaggcaaaaaagcagtcacataaaattctgcattttttaaaaatgttcaggatgaacagaagacatctttgtgcagaagaaatggtggagataccacgtgccgagaaaaagcaaaagaaaaagtaaaaagcaggaagggacacagctgtagctatttccatcaaagcaaaccactacttctgtgaccttcaaccaataaggaagtcaactttatgacacacgcaaagtgaccttgcaataccttacaattagtgggtcacaaaagtctattttaaaagaaaggcctcttgaattacccattctctgtgttttcagcattaaggactgtctgcaaaagcatgtccaaaagtgattgcatctgaaatggtaggctcttctaatttcgagtccaaatccataaggccaaaggttatcccaaagaccaccactcagacctccccaggactggccacgaccgacccgttgattgcttctcagtgcaccttggttaggagaccagtcacgttccatcctatcttcctgtggcctctgcaacgggagagccacaggatcccatgtaattgctgctttgctcctcagtaggttcagataggagagttctgatccccgccactcagcatgcttactgtgcctgacaaacttcaccacaaccgtccctttcatacagctgaagatggtgtttgtggaagctggaggtccctcttccttacagtactgcatttccgtgcccaagtgtgtttagaggacttaaaaacccaaatttcccaccctcccacccaaaacaaaacagaacaaaacaaaaaaaaagggggatgggggggacaaaaagaaaaaaaaaaaacaccctcatggggccctttatgcaaattatgtgcagtgccttttactttaaaattagttggcaaatgaccaagaccaacatctgaatattaacttttgctgaatagaaagacaaaaaaaccccactgtgactgggatgtggcaagttaaaatgggggagcaaaaagaggatacctctgagctatccatgaagatgggtttggacatggctcttttaaacacttcaatgtccctttgcaatcttttcaagttaaaaaaaaaatcagctttgccctcttgtagcggttcagtgtgttaatctcctcctgattcaagcagctttgcactttgtttttggaaaaaaaacaccacttctataaaaacacacaagaaacaaactcaagtttcaatgtagtcacgagctagctacaggactctgttgcacacaaactcctgtcatgggggactcttctctatcagccccttgcctcattgtcagatgtccttcagtcatgtaatgtgcaggacctgtattagcagaaaattggtatgttggatgtccagctatgccagtctcttggcggggattggagtagacggtcaaattaacgtccatagctccattctgtccaaagtccaaggtattagcagccactgggcgattctggtaggcctgattgccttggttaccagtagaggaggaagatgtcgaggaagaagtcgttgaggaagacagggatgtcatggagtggtgactgtggccaacctccatagaatcttgggtagaggagctattcgttggagaattgtagacccttggcctggtccggttacccaaggcttgttgtccatggtggtggtgatggtggtggtggtggtgatggtgatgggaactgttaccatggtgatgatgcaatgcattctgttgaggggctacatgaaaggttgtttcttgaacaggatgagtttcaacagtgacctgtgtaggagcttcagtgcctgaccaaccaagaggagcaggaaattgctgacgcacctggggactgtgtgtctcgcagtccatggcctgcacggcagctgtgaagtgcccaccactgtgccgatgctggtgcgtcggatccgaccgggctctcccactgttgcttgtccccgatgagccacctgagcttgacgatgtactggaggtggtgcccgaagactgagactgctccatggcggggcttgtagatacactattacttgtatttgtaccttcatcagctgttttcttgaagaaactgtgctgcagagcataataaggttgaattcgagttttggggtcataatcaagcatccttaaaatgaggtctttgaacttcaagtagtcagcgaccgtatgacctgactccccagcacgtcgcccaccaggtcctcctgtttccactccaagaatgttatgaagtttacgggttcctggtggtttgtactcccgttttccatctttggtcttctttaagttccaagtgccatctggcaacttctcaaagaactttcttgcttttggtgcttggtcaagaatatgagcaggtggaatacccagaacttccactattttattcatctgatctacctcattggcaccactgaacagaggttctccagtgtgcatttcaaccaaaatacacccgagggaccacatatcaatggcaaggtcataaggcattcccagtagcacctctggagaccgataaaagcgactctgaatatactggtatatcctctgccccaactgacaagaactgccaaagtcaactatcttgattgcactgcgtttggggttacaaagaaggatattttcaggttttagatcacagtgaatgatactaagttctggagtcgcaaggaaaagcagtgcagtgcacatctgttgcgcaaactttcgtgttaggttcaaagagacccctcggaaattggtgtttctcagcaagtcatagaggttgtaggacagcatttcaaaaactaaacagagatggtttcgaaacataaagtggcgtttcaaatgcactatgtagtatttcatttcagtgtcatgtttgttcatgagctcaagaagtcgcacttctatctgtgcttgattcagaaaagccttcttgttctttattattttaatggcaacccattcttgctccacacgatcatatgcctttacaacctgtccaaaggaacctttgcctatcaaggagtcaatttcgtaacgatccatccacttttctccgttttttacaatataatcatagttatcatcatcataaccatcattgtaaaccttccgttccttcttatgactagaatcgtctccctggccctgttggtgtcttcgcttcttttttgcatagtaaacctcattaatatgcttgtatgttttgatcaagtcaacagaaagttttctcaggggagcagttgctgggtcacggaaggtttggggcatccgcctctggttagttagaggttgctgaatctggtcagaatatgataaggcagaaacctgttggtcacttatgtttggctggcgacggtcactgtactgatgtgaatggggcatctgtccagccatctgaaggccagcagcatggaatgaaaatgacggtgcaagccgaacagatgaaggtttgcatgctgaagtctctcctcctgtatgcatcgtcttctttcaagtctcatatcatcctgatggggtgggggaagggagggaagagtccagcggcaaaactataacacgcggtccgggcgccgcgctcgcctctctccccgggaagcgcggcggccgcgaccgtccgcgcgtggagccggttcttcgaagggctggcgggcctcctagccggaaaatgcc

SEQ ID NO: 15206 - RNA, 14846 nt, Homo sapiens
  source 1..14846: mol_type = other RNA
gctgggattacaggcatgagccactgcacctggttgtattgtgttccttaggacagctaccatgtcattgcactttgctgcctaattcagtaacaattcatactccattgtaccttaaaagcacaatgatatttgaaatccacttttcttgtatatattggtaataaaaaataaaatgttgtagcatgggaatacaagtggcattcaaaatgctgctgagttataactgtgtcactgcaatttacattgcacagagcggcagggcaaaatgatgagaatgccacatattctcatcatacggtctctgcagcaactactcaattctgccacagtagcaccaaagtggccgtggacaacttgcaaatgaatgtggttatgttccaataaaacttcatttatggacactgaaattcaaatgtcatataatttccctatgtcctgaaatatcatttgatgtttttcagccatgtaaaatgtgaaaatcacccttagtttggtgagccatacaaaaacaggagggtaccttgctgatgcctaatctgcaatgggcaggaaacagaagccaaagtcgtccctgctcttccagagctctcctgttcctgaacagccgatagccctggaaggatgtgataacagcagcaggaaagcaggttgatgcttcagggagacaaaaactaaagcttccctcatagtcattagaacataatgaatctctcttattttttcttccatttacaaccctacttccacctttgttcagggtcctggagagcctcccagcttcttttaatcccggggcataatcctggggccccctctcacaaagaaaggggcctaaacgaaaattcatcagctgtgtgcagtggctcctgcccgtaatgggaggctgaggcagaaggatcgcttgagcccaggggttcaagaccagcatgggcaaaaaagtgcgacctcaactctacaaaatataaaataatttagccaggcacagtggcatgcgcctgtggtcccagctacttgggaggctgaggcaggaggatcgcctgagtcccagaggtggaggctgcagtaagcagagatcataccactgcactgcagcctgggcaacacagcaagaccctatccctaaaaaataatactaagaattgatgaagactaatctatgaagactaacatgtgggagaagcaagaggggactgtggaagccacatggggaagcacacactgtggagcgtcacccagcagtgtcccagcaccctggagctgctgctgctgcagacagcctgaaccagcagtggggaaagcggaagcagagcaggaactgtggatcctggaaacaagaaggggagaaaatgaccttgggaacagagaaatgggcaaagagcaggcttttgagaaggaaggaggaagcagcattgcatcactcagacttgattcttcagagcttcctggaagtgattctagtttcacaattaaacgagacgattgtcggagagaaacctgttcaacatctccaaattcatggacggttttgccaaaataaaaattttgtaggcaccagtgtggttcattaggacaatacaggcatccttcactacattttccctagccctaagcctagtgtctacattaattgatattaaattagtctcgcccctaaccctgcttctagtggtcacagcagctacagggaccatccagctgaaggtcttggtatgtgatctcgaaagtcaaggtcagcgtggagaactggaaagaggcctgactagaagacagactgtcgctggtcagttgtgtcatcttctgcaagttgcttaaacctgttaagttttctcactctaaagtgaggtgttggggcagtgtctctgactttgaatgtgcatgaatgacctggggaccttgttcaaatgcagattctcatccagtggtctgggctggggcctgagattttgcattgctagcaagcacccaggtgatgctaatgtcgtcagcccactgactacactgggcagcaaggggctggacaatcttctatcccttgatagatctaaaaaccatcctagggctgaggaagctgcaatgatgttaatttttagaacatacaagattctcttatttacgtatcctaggctgtcctcccaactccctctaggtcatccccttcgccatcagttgcctatatgagaatgaccagaaattggccattcccaggcccgactttcccctcctccatccattctttcagatgcctaccggacatctccacaacgttctcctacaagcccttagcactcaaagtcctcaaactctgggaggaagcctgactcctctcttttcacccctactcccagcatccattcagtccccgaggtctgtcagctctccttcctaaatagctctcgactctgtccacttataaactgatgctggcaagcctcctcaccttcgaatggcctgttgtcttctcctagattctagggcattcccaccaggataacacccattcctccattaggtatcagctagaacttcagttccttgggaatacagcacttcacagcctctctggattagaataaggtctctgttcacactcttttaaaaacactgggcttacttgtaattacttatctttcccacttataacaacaaaatgtgacatgctttttgtcctcatccctaagacctagctaagtgctttgcacatgactggtgttcaattaatatttgttgatttctcttatatagttctcacaccagctgtcccaagaccgtttgctggtaagacattcttcttcttcagggtaggactttttgttcatttttaaattgtttccagggttagtactgattgttttctttgattcagagtgtctctgcagggagtaggggagatatttcaagttcactgttttaattttgccagtaaaaggaaatttaccgttttgcttcttgcatctagtcactgctagccgcccccacttctagtgaagatggtcagaactctaatacgcaaacaaaaccgagctggggagaaagaccacaattagtgaatacgcacgtgggagccctccctggacaagctcctcatctgaattcttcaagactacagaagatgttaagtagctgtcattacataatcagtgggagatgccttcagaaacatccgcctacagaaagaggtagcccgtctctccagcacccacattcctgggcgagggtgacactccagtcagaaggtaagaatcccatgtaagcgctctgtgaagagcaaaccaccactcaattggaatacagtagcagtcctggaggaatccaggactccaagcgcactgagccctgtagatctcacccagcggtgagcgctggagcccctgctgggaggacccatcgtgccaaaggcctctgagcgcagagctgcccagactggccagggacaagacctggagctgctgggaagcacaaaagctcatccaatttacttctcccagaaatatcttatctacctgaagtgaacagttaaatcccatgattaggtcccttgtttcagcttcatcatccatccaaatccacggcccattgtaatgcaaatcatgtatagtctaatgcaaacaaacagacttttatcctaagacatttttgtccttatatttgatacaaggagaggatgatactttaggaataacaggctaatactgagagaacccaggctcgatgtagtcacctaatattatcaacaaagtcaacagaataaagaagaagaaaaaagcagcaattatttccttactgctttcaaaatgtgggttacaacctattacatttcaaaagcttccccgataatatccctgttttatttataaacttaagagctgatttctgtcaccctcatctcttcctatctacatcaaacctctgaaggctaaaaatgtaacagactttccttggagtgggagcaaagggtggggactggcccctggatgcgtgatcacaagggtctaatgaccatgcctgttcaaaaacagacccttaccacagttattcctccaggcagtctccctgaggttgtacagagaaattctactgaaaacccatccttataaaacatttaaatatcatatagtttatcaaggcaaagcaaactaccgaaaaactccctcacacctgtaatcccagcactttgggaggccaaggcagatggatcacaaggtcaggagactgagaccatcctgcctaacatggtgaaaccccatctctactaaaaatacacaaaaaaaattagccgggcgtggtggcgggcgccagtagtcccagctactctggaggctgaggcaggcgaatggcgtgaacccaggaggcggagcttgcagtgagccgagatcgcgccactgcactccagcctgggcgacagagcgagactccgcctcaaaaaaaaaaaaaaaaaaaaaaacttcccacaacaaacctcaaaactcttaaatagatgcagggactgtgcggtatgcaaaaccaactagtaaaggaatgttaacacctagtcccagactccaaaaataaaagtcagctggaaagcaatgctgtttagccctccacggagaacactgtccacctcatttccctgcattgtttgctgtatttacgtagaaaaagaagttccattcaggctgtggactccgctgtttagccgcatattatatttatcggacactttctacatactaggcattgtgctttctgcggacattacctcactgaggcatgcacagcatctcctaagtggacactataggtatctccattgtacaaagcggacagtaatccttgcgcaagttgagcagcgtacccagggtcacgaagccaatgagaggagcagtgggatctgaacctctttgggattctagagagggaaactgtaactactatacagagctggtggctggtgccctgggaaacccttcaccggcttacaagaccagatgagactgagatataaaggaactaattccattcccactgttgggaaataacatgtgccattctcatgggacatctgagagctattaatgaataggatgttacactgacccatctccacaagggaagacaacaaaaaggaacaaactgtgtaagttttatatacttacatctggcaatttctgcctttcccggaggcttgtttataacattttgtaatgcaccataaattgaaaattttaattatccattactctatgtaaactttggtaatcaaactccatttcaagatgttcttggggctgggtgaagtagctcacgcctgtaatcccagcactttgggaggccgaggcaggtggatagcttgaagtcgggagttcaagaccagcctggccaacattgcgaaaccccctctctatcaaaaatactattagctgggtgtggtggtgtgcacctgtaatcccagctacttgaaaggctgaggcacgagaatcgcttgaatctgggaaatggaggttgcagtgagccgagatcacacccctgcacaccaacctgggagacaaagcaagactgtctccaaaaaaaaaaaaaaaaaaagtccttggattcagacttccgtcatattagccacacgcctcttcttgccagagtcctgcctggctgcaggttcagaatggcccgcaaagtttcagaaaacagagctccaggccccaccccaactctgaatctaaaatcctgctagtgtgatggtcatccgtggttttataaagttctacagatgagtttagtgtgcagcaaggctggacagtcattttaaattgatgagtaccgattgagcagtttgcgatcactagagttcattagtcatttctttcctggatttgcgggcaatggaagtgggagtggtgcctgaagtgagctcctccccacctcgtggcatcacctcttcagcagaacaaggcttgtctgtgatgtacataaaaacgctctttctcatgctatttcactgcattccgcttttccgctttaaatctttacagacgtgagccaccacgcccagcctatttatgtttgagaggcccaggctggaggatcacttgaggccagcagtttgaggagcgcctgagcaactcagcaaaaccccgtattaaaaacagccaggcatggtggtgtgcacaggtagtcccagctacttgggaggctgagatgggaggatcacctagcccagttgtttaaggctgcagtgagctgcaatcacaccaccaaactccagcttgcgtgacaaagccagacaccgtctctaaaattaaagaagtaacattaaaaaaaacttagccgtttcatgccactagaggtattttctttcatttcagagggagttaacaaaccccaccccagcagtgcccttctctgcagtctttctgtccaacagtgagtggatgatgattccaaattcatcctcccagggtctcttttaagcaactcaacactttctgctggccacactcaggctcaggcccgtcctcttgcctgggtgttcattaacaactccctgcccggcacacctgcttggctgcttcctggccaccctagtgcagaactaccacacacacccagtgcctgccactttattttgcccttggctctgaatctcccgtgactgcagtttcagatatggaattcaggggcaagtacactgactaatgaatgagtatataatggaagcaaaactttacaagaataaagaaaaaaattcccaaagtagcaattttagaaatttaatcgggaagattatcaaatagctggtctttcagacagatgaaacattaagcacttatacctacacggcctttctctagctatgagaactcggccaaccacacccatgccagcatcgcccggcctcccatgcgaacagagctgggctccacttgtcttgtccacttgtttcctctgtcctgcatcatgaacttttgccaccactttgcctgacccaaacttaatgcactttattaatagtcaacatgactcaggctctagtactgtgctccttcaggacccagctgggactgaaccaggctacctggtaaaagcgaagggaagccggtttaagacttgtctctgcctcctctatgctttgaagaaggattcacaggttttgctggggatgacaggaaattcaactgaaatggaaatttacccacattaattccacacctgataacagggacataccctaaagatgggaaattatggggaaaaattttcaggtacagcagctgcatactggaagagagacctgtagcattctagttgtgtttcaaatcagcgtccagttggagaaacactttgtctcctaagatttaaagtaggaaattagaaataaatactgacaaatacctgacagtctcagtgttaaggtagtgttattttttttaaagttctgatgcaagaacacccactgagagcagccaaaatctgggaccttggctatgcataatgccaaagagagccaaacacaccaagcgatgagccacttacctcaatgaacatgtcttccacaaaacaagcatccagtgccttcaacacaggcatacgtcaaaaattcctggtccagggtgaaagcccagtaggcatccacaggctggttctcagtggattcatttggattaaggttagtcattaaaagggaggataacaaataagctatcttcttagggtttcttctcttgttctttgtactacaaattacttggtgatgtatgttttcacgcaaggaaacaggcctagataagaaaccagggttatgaaaatcagaacttctcctctactctccctgacaccaaaggttttccaacgtctggtcaacagacatccctagcagatttttaagaaatctgaatgaagtctgggtataccgaagtcacgcacggcttttgtccccattacattttcaaacttccttcatatatagcagtaagaccaagtcatgtatttggaatgaaccatctggtctattacatacagtctaccactataaaaatggacataaaaatgagtcttgaacttgtattctgtctatggggataccacccagaatgcaccggatcgcatctgaacctgcattctgcgactatcaaaataaaggcaggcccaaaggaaactgagaaactggcctagaactgagtgcctgctatctcgtcttcgtgtgtattttgattatgtatctccctattggaagaacagaaaagttcaacaccacaaaagctgggaagcagtacaggggcaaactcaatggtcacttgtgagcctaacataattactgaatctttcatgattttttacatgtagttttaaataaaaatgtcggtttttttttttcagcccaatatccatgtgcctaggtaaaattctcacaccctaagaagaaaactaatggaagttttcctttcttacatgtggttaacttcaactttacgcaaccaaccttaattttacagattcacgcttaacttttaaataagcatcttgcctctcgaaagccaccttaatatatactgaagcaggtgaatttgtaaaaagagaagactttaggttagcaattgaatcacagtggcaagaattctagaattctgatatggccccgtacgaggagttagggaaggaagaatgagtattcgtattccttccttcatccaagcacgtcaaagcatatcagagaaaaccatcagaccctcacatccagtcgaaatgctaccaactaaaatatgagcattttgaatcacaaaattatgtaaacattcaaataaaaaaatcaatgtgaaaaatcaaaatgatctgttaaacctccaatttttactttcagagattgctgatgcctatgtcaatgtatctcaaatagtttcctttttacacatttaactcaactttgatactatacctaccagacctggaccagtttaattgcataggaagatttttactatgtttacatttttcttaaattaatttttaaaaaagcatagtaaagagtctgaggacaaattattcaactgtttatcatacataagaccgcatgactataatacaaaggggggttcttttttcatttaacgttacaatatacacagcaagtccggactagatcttacaatctgaacacaggtatttaaccttttccatgctgtttatgtttacaatgcacagaagtcctgtaaccaaactgtgtagtaaagcacacaaaactggactgtaacataacacagtatgcagaagcattggattttatgattttctttacgtaaatatcggtttaaaaactgctttagttttttggtgcttgctaagatgtggcaaccagcacagaaaaaaaaaatgacctgacccatatgatatcttaaccttatattcctaaacagcagtaactactgaattccttttgatattgctatactcaagatgatatccttttattcactgtaaacctttatgaactaccaagttcaaaaaaatcatccacaggcttgacagttaattacaaaataaatatggatttcctgataaacaacaaaaagtttttgtagtttataaaaacgagtatttccaagtttccattcacatttacatagtgtttagcctttcttttctcactgtttacatataaaaacctgcttttgttcagaaaaaaaattgacctagtcagccacatggaattgaccaatagaatgaaacgcggtgttctgctgagtcatcttaaacaggttatcggcagaggtagattactgcttcttttctaggcttcttttgatcctggacaggtaaattacttatcttcattctcccaattcaaccgctcaaaagtgtcacaccccaaaattggtcaatttaaaatgggaacacaaatttagcaactgccagactgtgttacattaaggcagcgtaatctcaacacgaggcacctgttaaataccagcctgtctgctcaggtcacgcatgagagttctgctttgcttgcactcatactctggacctgttggtgcaatcaaggtcttgctttcaagtttacaagtaggttaatcaggaatacaagaatcaactgctggttccatagcttctggatccagtgtccctttaccttcagaagcctgaacacacttagaatgtaacagatgttgtaatcttgaattagatgtcaatctactatgttcagtacacagattgctgtaaatgtattggctatggattcaacaacagttccagttttgtttaagcaatagtacagccataattttcaactgacatttaaaaatggtctagttacaccttgtgtcaaagtgcagaactgctacattattggttacagacatctatgtgctataaaaacagctttggtacaataaattatcaaaaaagaaaataaatttttgtaaaattcacagcataattgtgaggcaaaaaagcagtcacataaaattctgcattttttaaaaatgttcaggatgaacagaagacatctttgtgcagaagaaatggtggagataccacgtgccgagaaaaagcaaaagaaaaagtaaaaagcaggaagggacacagctgtagctatttccatcaaagcaaaccactacttctgtgaccttcaaccaataaggaagtcaactttatgacacacgcaaagtgaccttgcaataccttacaattagtgggtcacaaaagtctattttaaaagaaaggcctcttgaattacccattctctgtgttttcagcattaaggactgtctgcaaaagcatgtccaaaagtgattgcatctgaaatggtaggctcttctaatttcgagtccaaatccataaggccaaaggttatcccaaagaccaccactcagacctccccaggactggccacgaccgacccgttgattgcttctcagtgcaccttggttaggagaccagtcacgttccatcctatcttcctgtggcctctgcaacgggagagccacaggatcccatgtaattgctgctttgctcctcagtaggttcagataggagagttctgatccccgccactcagcatgcttactgtgcctgacaaacttcaccacaaccgtccctttcatacagctgaagatggtgtttgtggaagctggaggtccctcttccttacagtactgcatttccgtgcccaagtgtgtttagaggacttaaaaacccaaatttcccaccctcccacccaaaacaaaacagaacaaaacaaaaaaaaagggggatgggggggacaaaaagaaaaaaaaaaaacaccctcatggggccctttatgcaaattatgtgcagtgccttttactttaaaattagttggcaaatgaccaagaccaacatctgaatattaacttttgctgaatagaaagacaaaaaaaccccactgtgactgggatgtggcaagttaaaatgggggagcaaaaagaggatacctctgagctatccatgaagatgggtttggacatggctcttttaaacacttcaatgtccctttgcaatcttttcaagttaaaaaaaaaatcagctttgccctcttgtagcggttcagtgtgttaatctcctcctgattcaagcagctttgcactttgtttttggaaaaaaaacaccacttctataaaaacacacaagaaacaaactcaagtttcaatgtagtcacgagctagctacaggactctgttgcacacaaactcctgtcatgggggactcttctctatcagccccttgcctcattgtcagatgtccttcagtcatgtaatgtgcaggacctgtattagcagaaaattggtatgttggatgtccagctatgccagtctcttggcggggattggagtagacggtcaaattaacgtccatagctccattctgtccaaagtccaaggtattagcagccactgggcgattctggtaggcctgattgccttggttaccagtagaggaggaagatgtcgaggaagaagtcgttgaggaagacagggatgtcatggagtggtgactgtggccaacctccatagaatcttgggtagaggagctattcgttggagaattgtagacccttggcctggtccggttacccaaggcttgttgtccatggtggtggtgatggtggtggtggtggtgatggtgatgggaactgttaccatggtgatgatgcaatgcattctgttgaggggctacatgaaaggttgtttcttgaacaggatgagtttcaacagtgacctgtgtaggagcttcagtgcctgaccaaccaagaggagcaggaaattgctgacgcacctggggactgtgtgtctcgcagtccatggcctgcacggcagctgtgaagtgcccaccactgtgccgatgctggtgcgtcggatccgaccgggctctcccactgttgcttgtccccgatgagccacctgagcttgacgatgtactggaggtggtgcccgaagactgagactgctccatggcggggcttgtagatacactattacttgtatttgtaccttcatcagctgttttcttgaagaaactgtgctgcagagcataataaggttgaattcgagttttggggtcataatcaagcatccttaaaatgaggtctttgaacttcaagtagtcagcgaccgtatgacctgactccccagcacgtcgcccaccaggtcctcctgtttccactccaagaatgttatgaagtttacgggttcctggtggtttgtactcccgttttccatctttggtcttctttaagttccaagtgccatctggcaacttctcaaagaactttcttgcttttggtgcttggtcaagaatatgagcaggtggaatacccagaacttccactattttattcatctgatctacctcattggcaccactgaacagaggttctccagtgtgcatttcaaccaaaatacacccgagggaccacatatcaatggcaaggtcataaggcattcccagtagcacctctggagaccgataaaagcgactctgaatatactggtatatcctctgccccaactgacaagaactgccaaagtcaactatcttgattgcactgcgtttggggttacaaagaaggatattttcaggttttagatcacagtgaatgatactaagttctggagtcgcaaggaaaagcagtgcagtgcacatctgttgcgcaaactttcgtgttaggttcaaagagacccctcggaaattggtgtttctcagcaagtcatagaggttgtaggacagcatttcaaaaactaaacagagatggtttcgaaacataaagtggcgtttcaaatgcactatgtagtatttcatttcagtgtcatgtttgttcatgagctcaagaagtcgcacttctatctgtgcttgattcagaaaagccttcttgttctttattattttaatggcaacccattcttgctccacacgatcatatgcctttacaacctgtccaaaggaacctttgcctatcaaggagtcaatttcgtaacgatccatccacttttctccgttttttacaatataatcatagttatcatcatcataaccatcattgtaaaccttccgttccttcttatgactagaatcgtctccctggccctgttggtgtcttcgcttcttttttgcatagtaaacctcattaatatgcttgtatgttttgatcaagtcaacagaaagttttctcaggggagcagttgctgggtcacggaaggtttggggcatccgcctctggttagttagaggttgctgaatctggtcagaatatgataaggcagaaacctgttggtcacttatgtttggctggcgacggtcactgtactgatgtgaatggggcatctgtccagccatctgaaggccagcagcatggaatgaaaatgacggtgcaagccgaacagatgaaggtttgcatgctgaagtctctcctcctgtatgcatcgtcttctttcaagtctcatatcatcctgatggggtgggggaagggagggaagagtccagcggcaaaactataacacgggacgatggcggggcgctcgcgccgcttcctccggtgagtctcagcctcgggctcccgcgccgcgctcccgccgcggcctccgcagccagcgccgccccggcagcctctctccgcccccggcgctccggctcctggccgcgccgcagcctgctcagtctctcctcggctcgcggttccagcggcgcccggggccggggaggcgacagccccctccccggcaaataccgcagtccccgggccccgattccaggcggcggggccgcacggccggcccggcgcagagggcggcgtcggcgaggccgggcgccgagcggcggctgctgccggcggcttcttcccgaggaggattttgtaaatctcacaaaatggcgcgcgctccgaacctgcgcagcgagaagcgccggggcccgggcggcggcggcggctcctccgccaggagagcccgaaccgcccgcccccgagtccccgcacagacagacagacactcgcacacacccgcacactcgcgcgcacaatcgccctcgcacacgctccctcgcacacacactcgcactcacaccggtcccgcctgctcgccggcggcggcagcggcaccaacagcagcagcaggaacagcagcagcagaagcggcggcggcggcgcccgcaccccccgctcggggtgtccgctctctgaggccgacctgggccgcgatcagcagcagcgacagcagcagtctccccggatacccccgccgcggttgccgccgccacccccgcctcactccaatggggctttttattattattcgggcgggaagcgaaagggtttaaaaaaaaaccaaccaacaaaatggcgacggaccgacccggtc

SEQ ID NO: 15207 - RNA, 14279 nt, Homo sapiens
  source 1..14279: mol_type = other RNA
gctgggattacaggcatgagccactgcacctggttgtattgtgttccttaggacagctaccatgtcattgcactttgctgcctaattcagtaacaattcatactccattgtaccttaaaagcacaatgatatttgaaatccacttttcttgtatatattggtaataaaaaataaaatgttgtagcatgggaatacaagtggcattcaaaatgctgctgagttataactgtgtcactgcaatttacattgcacagagcggcagggcaaaatgatgagaatgccacatattctcatcatacggtctctgcagcaactactcaattctgccacagtagcaccaaagtggccgtggacaacttgcaaatgaatgtggttatgttccaataaaacttcatttatggacactgaaattcaaatgtcatataatttccctatgtcctgaaatatcatttgatgtttttcagccatgtaaaatgtgaaaatcacccttagtttggtgagccatacaaaaacaggagggtaccttgctgatgcctaatctgcaatgggcaggaaacagaagccaaagtcgtccctgctcttccagagctctcctgttcctgaacagccgatagccctggaaggatgtgataacagcagcaggaaagcaggttgatgcttcagggagacaaaaactaaagcttccctcatagtcattagaacataatgaatctctcttattttttcttccatttacaaccctacttccacctttgttcagggtcctggagagcctcccagcttcttttaatcccggggcataatcctggggccccctctcacaaagaaaggggcctaaacgaaaattcatcagctgtgtgcagtggctcctgcccgtaatgggaggctgaggcagaaggatcgcttgagcccaggggttcaagaccagcatgggcaaaaaagtgcgacctcaactctacaaaatataaaataatttagccaggcacagtggcatgcgcctgtggtcccagctacttgggaggctgaggcaggaggatcgcctgagtcccagaggtggaggctgcagtaagcagagatcataccactgcactgcagcctgggcaacacagcaagaccctatccctaaaaaataatactaagaattgatgaagactaatctatgaagactaacatgtgggagaagcaagaggggactgtggaagccacatggggaagcacacactgtggagcgtcacccagcagtgtcccagcaccctggagctgctgctgctgcagacagcctgaaccagcagtggggaaagcggaagcagagcaggaactgtggatcctggaaacaagaaggggagaaaatgaccttgggaacagagaaatgggcaaagagcaggcttttgagaaggaaggaggaagcagcattgcatcactcagacttgattcttcagagcttcctggaagtgattctagtttcacaattaaacgagacgattgtcggagagaaacctgttcaacatctccaaattcatggacggttttgccaaaataaaaattttgtaggcaccagtgtggttcattaggacaatacaggcatccttcactacattttccctagccctaagcctagtgtctacattaattgatattaaattagtctcgcccctaaccctgcttctagtggtcacagcagctacagggaccatccagctgaaggtcttggtatgtgatctcgaaagtcaaggtcagcgtggagaactggaaagaggcctgactagaagacagactgtcgctggtcagttgtgtcatcttctgcaagttgcttaaacctgttaagttttctcactctaaagtgaggtgttggggcagtgtctctgactttgaatgtgcatgaatgacctggggaccttgttcaaatgcagattctcatccagtggtctgggctggggcctgagattttgcattgctagcaagcacccaggtgatgctaatgtcgtcagcccactgactacactgggcagcaaggggctggacaatcttctatcccttgatagatctaaaaaccatcctagggctgaggaagctgcaatgatgttaatttttagaacatacaagattctcttatttacgtatcctaggctgtcctcccaactccctctaggtcatccccttcgccatcagttgcctatatgagaatgaccagaaattggccattcccaggcccgactttcccctcctccatccattctttcagatgcctaccggacatctccacaacgttctcctacaagcccttagcactcaaagtcctcaaactctgggaggaagcctgactcctctcttttcacccctactcccagcatccattcagtccccgaggtctgtcagctctccttcctaaatagctctcgactctgtccacttataaactgatgctggcaagcctcctcaccttcgaatggcctgttgtcttctcctagattctagggcattcccaccaggataacacccattcctccattaggtatcagctagaacttcagttccttgggaatacagcacttcacagcctctctggattagaataaggtctctgttcacactcttttaaaaacactgggcttacttgtaattacttatctttcccacttataacaacaaaatgtgacatgctttttgtcctcatccctaagacctagctaagtgctttgcacatgactggtgttcaattaatatttgttgatttctcttatatagttctcacaccagctgtcccaagaccgtttgctggtaagacattcttcttcttcagggtaggactttttgttcatttttaaattgtttccagggttagtactgattgttttctttgattcagagtgtctctgcagggagtaggggagatatttcaagttcactgttttaattttgccagtaaaaggaaatttaccgttttgcttcttgcatctagtcactgctagccgcccccacttctagtgaagatggtcagaactctaatacgcaaacaaaaccgagctggggagaaagaccacaattagtgaatacgcacgtgggagccctccctggacaagctcctcatctgaattcttcaagactacagaagatgttaagtagctgtcattacataatcagtgggagatgccttcagaaacatccgcctacagaaagaggtagcccgtctctccagcacccacattcctgggcgagggtgacactccagtcagaaggtaagaatcccatgtaagcgctctgtgaagagcaaaccaccactcaattggaatacagtagcagtcctggaggaatccaggactccaagcgcactgagccctgtagatctcacccagcggtgagcgctggagcccctgctgggaggacccatcgtgccaaaggcctctgagcgcagagctgcccagactggccagggacaagacctggagctgctgggaagcacaaaagctcatccaatttacttctcccagaaatatcttatctacctgaagtgaacagttaaatcccatgattaggtcccttgtttcagcttcatcatccatccaaatccacggcccattgtaatgcaaatcatgtatagtctaatgcaaacaaacagacttttatcctaagacatttttgtccttatatttgatacaaggagaggatgatactttaggaataacaggctaatactgagagaacccaggctcgatgtagtcacctaatattatcaacaaagtcaacagaataaagaagaagaaaaaagcagcaattatttccttactgctttcaaaatgtgggttacaacctattacatttcaaaagcttccccgataatatccctgttttatttataaacttaagagctgatttctgtcaccctcatctcttcctatctacatcaaacctctgaaggctaaaaatgtaacagactttccttggagtgggagcaaagggtggggactggcccctggatgcgtgatcacaagggtctaatgaccatgcctgttcaaaaacagacccttaccacagttattcctccaggcagtctccctgaggttgtacagagaaattctactgaaaacccatccttataaaacatttaaatatcatatagtttatcaaggcaaagcaaactaccgaaaaactccctcacacctgtaatcccagcactttgggaggccaaggcagatggatcacaaggtcaggagactgagaccatcctgcctaacatggtgaaaccccatctctactaaaaatacacaaaaaaaattagccgggcgtggtggcgggcgccagtagtcccagctactctggaggctgaggcaggcgaatggcgtgaacccaggaggcggagcttgcagtgagccgagatcgcgccactgcactccagcctgggcgacagagcgagactccgcctcaaaaaaaaaaaaaaaaaaaaaaacttcccacaacaaacctcaaaactcttaaatagatgcagggactgtgcggtatgcaaaaccaactagtaaaggaatgttaacacctagtcccagactccaaaaataaaagtcagctggaaagcaatgctgtttagccctccacggagaacactgtccacctcatttccctgcattgtttgctgtatttacgtagaaaaagaagttccattcaggctgtggactccgctgtttagccgcatattatatttatcggacactttctacatactaggcattgtgctttctgcggacattacctcactgaggcatgcacagcatctcctaagtggacactataggtatctccattgtacaaagcggacagtaatccttgcgcaagttgagcagcgtacccagggtcacgaagccaatgagaggagcagtgggatctgaacctctttgggattctagagagggaaactgtaactactatacagagctggtggctggtgccctgggaaacccttcaccggcttacaagaccagatgagactgagatataaaggaactaattccattcccactgttgggaaataacatgtgccattctcatgggacatctgagagctattaatgaataggatgttacactgacccatctccacaagggaagacaacaaaaaggaacaaactgtgtaagttttatatacttacatctggcaatttctgcctttcccggaggcttgtttataacattttgtaatgcaccataaattgaaaattttaattatccattactctatgtaaactttggtaatcaaactccatttcaagatgttcttggggctgggtgaagtagctcacgcctgtaatcccagcactttgggaggccgaggcaggtggatagcttgaagtcgggagttcaagaccagcctggccaacattgcgaaaccccctctctatcaaaaatactattagctgggtgtggtggtgtgcacctgtaatcccagctacttgaaaggctgaggcacgagaatcgcttgaatctgggaaatggaggttgcagtgagccgagatcacacccctgcacaccaacctgggagacaaagcaagactgtctccaaaaaaaaaaaaaaaaaaagtccttggattcagacttccgtcatattagccacacgcctcttcttgccagagtcctgcctggctgcaggttcagaatggcccgcaaagtttcagaaaacagagctccaggccccaccccaactctgaatctaaaatcctgctagtgtgatggtcatccgtggttttataaagttctacagatgagtttagtgtgcagcaaggctggacagtcattttaaattgatgagtaccgattgagcagtttgcgatcactagagttcattagtcatttctttcctggatttgcgggcaatggaagtgggagtggtgcctgaagtgagctcctccccacctcgtggcatcacctcttcagcagaacaaggcttgtctgtgatgtacataaaaacgctctttctcatgctatttcactgcattccgcttttccgctttaaatctttacagacgtgagccaccacgcccagcctatttatgtttgagaggcccaggctggaggatcacttgaggccagcagtttgaggagcgcctgagcaactcagcaaaaccccgtattaaaaacagccaggcatggtggtgtgcacaggtagtcccagctacttgggaggctgagatgggaggatcacctagcccagttgtttaaggctgcagtgagctgcaatcacaccaccaaactccagcttgcgtgacaaagccagacaccgtctctaaaattaaagaagtaacattaaaaaaaacttagccgtttcatgccactagaggtattttctttcatttcagagggagttaacaaaccccaccccagcagtgcccttctctgcagtctttctgtccaacagtgagtggatgatgattccaaattcatcctcccagggtctcttttaagcaactcaacactttctgctggccacactcaggctcaggcccgtcctcttgcctgggtgttcattaacaactccctgcccggcacacctgcttggctgcttcctggccaccctagtgcagaactaccacacacacccagtgcctgccactttattttgcccttggctctgaatctcccgtgactgcagtttcagatatggaattcaggggcaagtacactgactaatgaatgagtatataatggaagcaaaactttacaagaataaagaaaaaaattcccaaagtagcaattttagaaatttaatcgggaagattatcaaatagctggtctttcagacagatgaaacattaagcacttatacctacacggcctttctctagctatgagaactcggccaaccacacccatgccagcatcgcccggcctcccatgcgaacagagctgggctccacttgtcttgtccacttgtttcctctgtcctgcatcatgaacttttgccaccactttgcctgacccaaacttaatgcactttattaatagtcaacatgactcaggctctagtactgtgctccttcaggacccagctgggactgaaccaggctacctggtaaaagcgaagggaagccggtttaagacttgtctctgcctcctctatgctttgaagaaggattcacaggttttgctggggatgacaggaaattcaactgaaatggaaatttacccacattaattccacacctgataacagggacataccctaaagatgggaaattatggggaaaaattttcaggtacagcagctgcatactggaagagagacctgtagcattctagttgtgtttcaaatcagcgtccagttggagaaacactttgtctcctaagatttaaagtaggaaattagaaataaatactgacaaatacctgacagtctcagtgttaaggtagtgttattttttttaaagttctgatgcaagaacacccactgagagcagccaaaatctgggaccttggctatgcataatgccaaagagagccaaacacaccaagcgatgagccacttacctcaatgaacatgtcttccacaaaacaagcatccagtgccttcaacacaggcatacgtcaaaaattcctggtccagggtgaaagcccagtaggcatccacaggctggttctcagtggattcatttggattaaggttagtcattaaaagggaggataacaaataagctatcttcttagggtttcttctcttgttctttgtactacaaattacttggtgatgtatgttttcacgcaaggaaacaggcctagataagaaaccagggttatgaaaatcagaacttctcctctactctccctgacaccaaaggttttccaacgtctggtcaacagacatccctagcagatttttaagaaatctgaatgaagtctgggtataccgaagtcacgcacggcttttgtccccattacattttcaaacttccttcatatatagcagtaagaccaagtcatgtatttggaatgaaccatctggtctattacatacagtctaccactataaaaatggacataaaaatgagtcttgaacttgtattctgtctatggggataccacccagaatgcaccggatcgcatctgaacctgcattctgcgactatcaaaataaaggcaggcccaaaggaaactgagaaactggcctagaactgagtgcctgctatctcgtcttcgtgtgtattttgattatgtatctccctattggaagaacagaaaagttcaacaccacaaaagctgggaagcagtacaggggcaaactcaatggtcacttgtgagcctaacataattactgaatctttcatgattttttacatgtagttttaaataaaaatgtcggtttttttttttcagcccaatatccatgtgcctaggtaaaattctcacaccctaagaagaaaactaatggaagttttcctttcttacatgtggttaacttcaactttacgcaaccaaccttaattttacagattcacgcttaacttttaaataagcatcttgcctctcgaaagccaccttaatatatactgaagcaggtgaatttgtaaaaagagaagactttaggttagcaattgaatcacagtggcaagaattctagaattctgatatggccccgtacgaggagttagggaaggaagaatgagtattcgtattccttccttcatccaagcacgtcaaagcatatcagagaaaaccatcagaccctcacatccagtcgaaatgctaccaactaaaatatgagcattttgaatcacaaaattatgtaaacattcaaataaaaaaatcaatgtgaaaaatcaaaatgatctgttaaacctccaatttttactttcagagattgctgatgcctatgtcaatgtatctcaaatagtttcctttttacacatttaactcaactttgatactatacctaccagacctggaccagtttaattgcataggaagatttttactatgtttacatttttcttaaattaatttttaaaaaagcatagtaaagagtctgaggacaaattattcaactgtttatcatacataagaccgcatgactataatacaaaggggggttcttttttcatttaacgttacaatatacacagcaagtccggactagatcttacaatctgaacacaggtatttaaccttttccatgctgtttatgtttacaatgcacagaagtcctgtaaccaaactgtgtagtaaagcacacaaaactggactgtaacataacacagtatgcagaagcattggattttatgattttctttacgtaaatatcggtttaaaaactgctttagttttttggtgcttgctaagatgtggcaaccagcacagaaaaaaaaaatgacctgacccatatgatatcttaaccttatattcctaaacagcagtaactactgaattccttttgatattgctatactcaagatgatatccttttattcactgtaaacctttatgaactaccaagttcaaaaaaatcatccacaggcttgacagttaattacaaaataaatatggatttcctgataaacaacaaaaagtttttgtagtttataaaaacgagtatttccaagtttccattcacatttacatagtgtttagcctttcttttctcactgtttacatataaaaacctgcttttgttcagaaaaaaaattgacctagtcagccacatggaattgaccaatagaatgaaacgcggtgttctgctgagtcatcttaaacaggttatcggcagaggtagattactgcttcttttctaggcttcttttgatcctggacaggtaaattacttatcttcattctcccaattcaaccgctcaaaagtgtcacaccccaaaattggtcaatttaaaatgggaacacaaatttagcaactgccagactgtgttacattaaggcagcgtaatctcaacacgaggcacctgttaaataccagcctgtctgctcaggtcacgcatgagagttctgctttgcttgcactcatactctggacctgttggtgcaatcaaggtcttgctttcaagtttacaagtaggttaatcaggaatacaagaatcaactgctggttccatagcttctggatccagtgtccctttaccttcagaagcctgaacacacttagaatgtaacagatgttgtaatcttgaattagatgtcaatctactatgttcagtacacagattgctgtaaatgtattggctatggattcaacaacagttccagttttgtttaagcaatagtacagccataattttcaactgacatttaaaaatggtctagttacaccttgtgtcaaagtgcagaactgctacattattggttacagacatctatgtgctataaaaacagctttggtacaataaattatcaaaaaagaaaataaatttttgtaaaattcacagcataattgtgaggcaaaaaagcagtcacataaaattctgcattttttaaaaatgttcaggatgaacagaagacatctttgtgcagaagaaatggtggagataccacgtgccgagaaaaagcaaaagaaaaagtaaaaagcaggaagggacacagctgtagctatttccatcaaagcaaaccactacttctgtgaccttcaaccaataaggaagtcaactttatgacacacgcaaagtgaccttgcaataccttacaattagtgggtcacaaaagtctattttaaaagaaaggcctcttgaattacccattctctgtgttttcagcattaaggactgtctgcaaaagcatgtccaaaagtgattgcatctgaaatggtaggctcttctaatttcgagtccaaatccataaggccaaaggttatcccaaagaccaccactcagacctccccaggactggccacgaccgacccgttgattgcttctcagtgcaccttggttaggagaccagtcacgttccatcctatcttcctgtggcctctgcaacgggagagccacaggatcccatgtaattgctgctttgctcctcagtaggttcagataggagagttctgatccccgccactcagcatgcttactgtgcctgacaaacttcaccacaaccgtccctttcatacagctgaagatggtgtttgtggaagctggaggtccctcttccttacagtactgcatttccgtgcccaagtgtgtttagaggacttaaaaacccaaatttcccaccctcccacccaaaacaaaacagaacaaaacaaaaaaaaagggggatgggggggacaaaaagaaaaaaaaaaaacaccctcatggggccctttatgcaaattatgtgcagtgccttttactttaaaattagttggcaaatgaccaagaccaacatctgaatattaacttttgctgaatagaaagacaaaaaaaccccactgtgactgggatgtggcaagttaaaatgggggagcaaaaagaggatacctctgagctatccatgaagatgggtttggacatggctcttttaaacacttcaatgtccctttgcaatcttttcaagttaaaaaaaaaatcagctttgccctcttgtagcggttcagtgtgttaatctcctcctgattcaagcagctttgcactttgtttttggaaaaaaaacaccacttctataaaaacacacaagaaacaaactcaagtttcaatgtagtcacgagctagctacaggactctgttgcacacaaactcctgtcatgggggactcttctctatcagccccttgcctcattgtcagatgtccttcagtcatgtaatgtgcaggacctgtattagcagaaaattggtatgttggatgtccagctatgccagtctcttggcggggattggagtagacggtcaaattaacgtccatagctccattctgtccaaagtccaaggtattagcagccactgggcgattctggtaggcctgattgccttggttaccagtagaggaggaagatgtcgaggaagaagtcgttgaggaagacagggatgtcatggagtggtgactgtggccaacctccatagaatcttgggtagaggagctattcgttggagaattgtagacccttggcctggtccggttacccaaggcttgttgtccatggtggtggtgatggtggtggtggtggtgatggtgatgggaactgttaccatggtgatgatgcaatgcattctgttgaggggctacatgaaaggttgtttcttgaacaggatgagtttcaacagtgacctgtgtaggagcttcagtgcctgaccaaccaagaggagcaggaaattgctgacgcacctggggactgtgtgtctcgcagtccatggcctgcacggcagctgtgaagtgcccaccactgtgccgatgctggtgcgtcggatccgaccgggctctcccactgttgcttgtccccgatgagccacctgagcttgacgatgtactggaggtggtgcccgaagactgagactgctccatggcggggcttgtagatacactattacttgtatttgtaccttcatcagctgttttcttgaagaaactgtgctgcagagcataataaggttgaattcgagttttggggtcataatcaagcatccttaaaatgaggtctttgaacttcaagtagtcagcgaccgtatgacctgactccccagcacgtcgcccaccaggtcctcctgtttccactccaagaatgttatgaagtttacgggttcctggtggtttgtactcccgttttccatctttggtcttctttaagttccaagtgccatctggcaacttctcaaagaactttcttgcttttggtgcttggtcaagaatatgagcaggtggaatacccagaacttccactattttattcatctgatctacctcattggcaccactgaacagaggttctccagtgtgcatttcaaccaaaatacacccgagggaccacatatcaatggcaaggtcataaggcattcccagtagcacctctggagaccgataaaagcgactctgaatatactggtatatcctctgccccaactgacaagaactgccaaagtcaactatcttgattgcactgcgtttggggttacaaagaaggatattttcaggttttagatcacagtgaatgatactaagttctggagtcgcaaggaaaagcagtgcagtgcacatctgttgcgcaaactttcgtgttaggttcaaagagacccctcggaaattggtgtttctcagcaagtcatagaggttgtaggacagcatttcaaaaactaaacagagatggtttcgaaacataaagtggcgtttcaaatgcactatgtagtatttcatttcagtgtcatgtttgttcatgagctcaagaagtcgcacttctatctgtgcttgattcagaaaagccttcttgttctttattattttaatggcaacccattcttgctccacacgatcatatgcctttacaacctgtccaaaggaacctttgcctatcaaggagtcaatttcgtaacgatccatccacttttctccgttttttacaatataatcatagttatcatcatcataaccatcattgtaaaccttccgttccttcttatgactagaatcgtctccctggccctgttggtgtcttcgcttcttttttgcatagtaaacctcattaatatgcttgtatgttttgatcaagtcaacagaaagttttctcaggggagcagttgctgggtcacggaaggtttggggcatccgcctctgtaacatgacaatatcaggcatcacctggttagttagaggttgctgaatctggtcagaatatgataaggcagaaacctgttggtcacttatgtttggctggcgacggtcactgtactgatgtgaatggggcatctgtccagccatctgaaggccagcagcatggaatgaaaatgacggtgcaagccgaacagatgaaggtttgcatgctgaagtctctcctcctgtatgcatcgtcttctttcaagtctcatatcatcctgatggggtgggggaagggagggaagagtccagcggcaaaactataacactttcggggcgcagcctgcctgctccatcggaatgccctttagatgaatccccttgtgctgttactgtgtccttgtcgtccagctctctggttttcttttctatacaccttctcggtttccagagtcttaattcgcctgcttgtccttaaccatcaaaactctttattaatatcctggctttcgctgatttttattctccctaccccttctccctagctatgtattgctgggtgagctcccgaggcttgaaaacccaagtat

SEQ ID NO: 15208 - RNA, 17993 nt, Homo sapiens
  source 1..17993: mol_type = other RNA
gctgggattacaggcatgagccactgcacgtggctacatgttttgtatttttagtagagacggggtttcaccatgttggccaggctggtctcgaactcctgacctcaagtgatccacctgcctcagcctcccaaagtgctgagattacaggcgttgagccaccatgcccagcccttgaaatttaaatttcaatgtctctaaatgaagttttattggaacacatctacactcatttgtgtgtgtgtgtctgtgtgtgtgtgtgtgtgtgtgtgtgtgtgtgtgtggatggagatagagagagagggatttatgaatttatgataaggaattggcttatagaattaaggaggctggcaagtcccaaatcttcagggtggatgagcaggctggagaaccaggagaatacatattccagtgagagcccagtggcacctgctgtggagcaggattagtagatggtgtgcatgaactctgaaggcagtctgcggaagaattctctcttgcctgagagagagtctggggcagccagactttatgttctcctcaggtcttcaggtgattggatgaagcccacccacagatagagggcaatctgctttcctcaaagtccacaaatttaaacgttaatctcatccaaagcaacctcacagaaacacccagcataatgtttgatcaaatacctggggaccttgtggctcagccaagttgacacctaaaatttaccctcacactccagtcctccaacatcccagcttccctcttacatccctgaatggcagaacccaacaaggaaccagctggcgaagcagcatcgtgcctgttctttgttgcctgtgtttttcattttaagtcggtggagttacaacccatggattcctttgtgtctgcttccttttcattaaaattctgctcatggattcatccctgcagtaggttcattttcaggtggaagtgtaggaagcacaggagatcacagaagacctcagcaggccagctttgcaacatcctaacaaggagacgggaaactgaagtaccacaggaaggagatactctccatctctcaccacccaaagcttcctgggatgctaagggtcatcgttctttttttttttttttcccgctctgttgtccaggctggagtgcagtggcactatctcggctcaccacaacgtccgcctcccaggttcaaacgattctcctgtctcagcctccccagtagctgggatttacaggtgcccgctaccacgcctggctacttttgtatttttagtagagacagggagttcagactggtctcgaactcccgttctcaggtgatctgcccacctcagcctcccaaagtgttgggattacaggtgtgagccaccgtgcctggcctaagcctcactgttcttttcatctttcctgctgagacaggagattgaggatgtggacattttgttgaggaaagaaataggacagacaactcaatgaagtctcagagagccattctaagaacccatgttctatttccagaacccacgtcaggccattactggggggtctgatggggttatgagagaaatgcccagggagggagactggagaaggttcagggaccaagttctggcttctgcccttagaggagccggacctgcagagagagagtgggaaagtggagaaccatcagctcactttccctcacgccatggcaaaagcatctccatcaggcaggactggcttcacaggcaggcagcctgggcagccctgcggggccccacacttagaatggcctccgcctgctatcttgctctgctgtcagggtcttgaaattctgaatggtcttgaacatcatgcactgcacctggcaaaatagccggtcctgatcaggtctcaaggcagccctggactttggaaggcagcactgacgccccactgaggaaaggaatggctgctgaggactgagaactagagctgagactcccaggcagcccctttggaaaacagtttggcatttccccaaaatgttaaatgtggaattatgtgattcagaaaatcacatacaaaattgtctcgtgtcccttttaaacatatagaatgtaactattggaaagagagagaaaaagggcctggcttggtggctcacttctgtaatcccagcactttgggaggctgaggtgggcagatcacttgaggtcaagagttcaagaccaagctggctaacatggtgaaaccctgcctttaccaaaaaaaaaaaaaaaaaaattagccgggcgtggtggcgcacacctgtagtcccaacaggctgaggaagcagcttcacttgtacccaggaggtgcaggttgcagtgagccaagattgcctccactccagctcgagctacagagtgagactctgtctcaaaaaagaaaaaaaaaagagagaaagaagttttggaaacattatttgcccttagccatgttgtgggtttatttcctacactgagtcatattatgtgtcttccaacatgtctggagcagttgctactccctgtacaccaggtccagtgactataatgtcatcaatataatggaccagtgtgtcgtcctgagggtgaaaaggttctcaaaggacctgggaactagatcatgagctgggcggcagagttgaggcagccttgagatagggtggtgaaggtgtatctagctgaaagcaaactgttcctgatggtctttactcacaggtatagagaaacattcaccagatgggtaactgggcagccaaggggataatcggatcgggtgtgccacacttcgcctgccccgcttgcttttggttgcttgctctttgttattttttcccccatgaagctgaaggccacgatagctgaaggctatgctattgaacactgtaactcaacttttacgtgctaccttatagataacatttataagtcaccataacaaccacttatttttcaggaacttggggcagatcctgtccagttcaaaccagttgagactgccaacccttcaactgggcctgtacacatgcccaagaggtggccttttgacatcagagggccaaaaactccaccctcagatcatgttaacgccaccattttctgcacatatgtcatatgaaccccaattatgactgcatttttccccactgccaatcacctttccccatgcctcagaccaccctacttctctaacctataaatctctctaagcctcatctttggggaggtgaatttgagagccattctcccatctcctcactggacagccttgtgaataattcttctctcttttgcaaaacccatgtcacagtgattgatttactgtgtgagaacagaacaaacctgggcctggctcagtaacaactgcaaaccagttgtcagacgtatcgtttgctcagcactgaaaccacatgtggaaacagcacctgcacttggaatcactagttaattaagtttacaattaatccaattgtcattctccaagatccatctgtcttctgcacaggctgagtaggtgagctaagtggagatgtgttcccgtctttgatggtggcactaatctcaacaatctctccaggaatgtggtattagtttgctttaatatttttgtgaatgaggcagctctagtggcttctacttggccttttctaccagaattacttttactgtatggatcagggaactagtgtgggattctgcccattgttgactatgtctattctaattacgcattctagaaccagggaaataaccataggatgggttcaggaatctactagatctactgtgagatgaatctgagccaaaaagcccattgatcacctgacctccatacactcttactctgaggaaccatggtggcattttgagtctcctgtaattactgctagttcagaactagaggctggttatcccagaaaagtctaattatttgcccttcccaatgcacaatcactctgataaatggccttgggtgcctttggggaggcctaggaagataaaaagtataaattattgtcagtgcagcagggtcctacttcaaagggacctggcctatcctttattcaagaagctgtgggtttgtgaactagatcaagacttggaattgactgagtgattgtaactctgtgttggtaatttaggtcagactttattcaccagatctggagctttcctacttactcggatcaagtaaaactttagtaggcagcccatccatttcagttctcaggacactatgatcagcaggcagacatcacagatctctgtgggtcagaccattcaggatcctgctttggctgcactgtccatggcagtcaccacaccaattgtgtttttggtgactaagtgttaccatatggtccctgcctcctcaggattccatcagccccactgcacttcagggagcatttcccactgtaatgtggcctgtatagaatatctggcactctctacatgaatttatttctcataatgaagtgtcctctggaccctccctgggtgggtgagcaggtatttacatgataaatactcaagcatttttatctccttaagcatttacatatcttcctctacagtataccaacgaagttctcgcatttcaactcattcagtgcaggttatgtttgcattcgtgttttttttttcttttggagatgagttctcactatattgcccaagccagtctcaaactcctggcctcaagcaatcctcccacctcagcctcccaagctgggattacagtgagtccatatctcaacaactcaaagcaaatgaagacagccattctcagcttctcaagttaaaacaatgaaccacaaatctctgcttaattatcccatatcgaataattcagcttgatctgactttatattccttccacgatgatcctgcacccttgttaccgcaaaaggttcccaatccagaccccaagagagggttcttggatctcgcacaagaaagaattcagggcgagtccgtaaagagaaagcaagtttattaagtaaaggaataaaagaatggctactccatagacagagcagccccgagggctgctggttgtctattttatggtttcttgatgatatgctaaacaaggggtggattattcatgcctcccctctccaggccatatagggtaacttcctgatgttgccatggcaactgtaaactgtcatggcactggtgggagggtagcagtgaggatgaccagaggtcattctcatcaccgtcttggttttggtgggttttagctggcttctttactgcaacctgctttatcagcaaggtctttgtggcctggatcttgtgccaatctcctatctcatcccgtgacttagaatgccttaaccgtctgggaatgcagcccagtaggtctcagcctcattttgttacaggaaaggggtcccgatccagactcttaagagagttcttggatctcgtgcaagaaaggattcagggcaagtccgcagtgcaaagcaaaaacaagtttattaagaaagtaaagtggtgaaaggacagctactccatagagtaggatggagtaacctctaacctgaggtcagtcaagtgtccttgccttttattaagaggggcctctaactcactctgtcttaggagaaactccaactcccctaagttgggcctctaacccaatcccatttgttactcgggtaccccatcacttacccaaagtcgtccaatcagtgctgcagtctatttctttggggttggggggatttcttcagtatcatcctttctgtggtttgccagaaatatgttacaggaccccaacacttacgcaaaggtagccgttgggtcaacgtttctgcactatagtcccttctgtggtcaccagaaatatgttacaggaaaggggtcccaattcaatcctagagggtaggaatgcctaactttctgagaatgcaggccagtaagtctcagcctcattttcccagccctcactcaaaatggagtcgctctggttcaaatacctctgacacttttacccagcccctattcaacatggagttgctctcgttccaatgcttctgacgctatctctacagattccccaggtttctataaaaattggcaaaattatgcaatttggagagtactgtatctcctcagtcacattttgcacttcacttttttttttttttaattgagacaaagtttcactctgtcgcccaggctggagtgcagttgtgcgatctcggctcactgcaacttccacctcctgggttcaagtgattctcctgcctcagcctccccagtagctaggattacaggcacacaccaccacacccggctaatttttgtatttttaatagagatggggtttcaccatattggccaggctggctggtctcaatctcctgatctcgtgatctgcccgcctcagcctcccgagtagctgggactacaggcgcccgctgccacgcccggttaattttttgtatttttactagagacggggtttcaccgcgttagccagcatggtctcgatctcttgacctcgtgatctgcccgcctcagcctcccaaagtgctgggattacaggtgtgagccaccgtgcctggccaaaaaaataatttttttaaaaggactccaggcaatgatagactggattaagaaaatgtggcacacatacaccatggaatactatgcagccataaaaaatgatgagttcatgtcctttgtagggacatggatgaaggtggaaataatcattctcagtaaactatcgcaagaacaaaaaaccaaacaccgcatattctcactcataggtgggaattgaacaatgagaaaacatggacacaggaaggggaacatcacactctggggactgttgtggggtggggggagggggggagggatagcattgggagatatacctaatgctagatgatgagttagtgggtgcagcgcaccagcatggcacatgtatacatatgtaactaacctgcacattgtgcacatgtaccctaaaagtataaaaaaaaaaaaaacaaggactccaggcatggtggctcacacctgtaatcccagcactttggcaagctgaggcaggtgggtcacttgaggtcaggagttcaagaccagcttgggcaacatggccaaaccttgtctctacaaaaatacaaaaattagctgggtgtggtggtgcacgcttgtagtcccagctagtcaggaggctgaggctggagaatcgcttgagcctgggaaagtggaggttgcagtgagctgagatcgtgccactgcactccagcctgggtgacagggtgagaccttgtctcaaaaaaaaaaaaaaaaaaaaagcaaaacgcaaaaagcagtggtgaccataggtcatgagcaacgtcagcggacttttggaagacatatacctcagggaaggccattacatgttcttcaggcaaaaggtggttaactaacactcaaagtctcattgtgaccctcccttctgctccctgccccagcattagtagctgggacctctccacagaagcacagatccaaaggccacagggcccctccctgagcacagacactatgtcagcccagcagtccactcctccaccataggtctgagttcagctccacaaggtccctcttccaatctcccacctttcaacaattctagccacgtctctttgttcctgctttgcactttgctccacatgaggtgggatcaataaactaccatcactcaaaactggttcggatgttgaaactgatgacactgcagacaccaagaggttatgaaaaagtttactactcacatgaggccttctagggaaagcaaagcgggcacccacgccagtctgttgggcttcagtgaaaggacgaacaagtggctctggtttttgttgtggttatgagagctcagtgcatttgacagtcagggtttgcacagtttgaacttcccctctgacgcaaagaggaagtggctgggctttcttatcagcttgtccagatccaggcaaactgagggggagagcttgaatgctattagcagacaaacgtcaaacatggggagactctattctagctcccccagtcctggggtggcagctgcttagcagttgctacctccaagacaccttggcattttcttcttgcctttttagctacttaaatatagtacacttctttataaggtctttgctaaaataactggtgtggtttctggcaactaaaacctggctgatataaaatctccttgctgttcttagcagggttaacattaactttaaaaggtgtggtagctggcatacaagtatttactctccttttcctcatctaataaagtagaatgaaaaacatctccatcttctggatcccatttcttcattaaaattatgagtttacagcttctggcttcacttgttatttattaagcaaaattaaggagatttaggcaaggaggagcttataatttcctataaagtgcatgtcttggtgactgtgcgtcagtatatagagaacatcctcatttttaaaaaaactgtggcctggtatttcatcatagatgtactagagttacttaagcgttcgtttactaatagccatttgtattgctcctgttaccagaaagcggtcgtgatccagtccccaagagagagttcttggaccttgctcaagaaaagaattcgggcgagtccacaaagtgaaagtagttaatattaagaaagtaaagaaatacagaatggctactccataggaagagtagccccaagggctgctggttgcctatttttatggttatttattgattatatgctaaacaaggggtagattattcataagtttcccgggaaaggtgtgagcaattaccagaactgagggttcctctcctttttagaccatatagtgttacttcctgatgttgccatggcattttttttttttttttttgagacagagtcttgctctgtcacccaggctggagtgcagtggcaccatcttggctcactgcaacctccaactcccgggatctagagattctcctgcctcagcctctcaagtagctgggattacaggcacgtgccaccatgcccagctaatttttgtattttttagtagagacagggtttcaccatgttggccaggctggtctcaatctcctgacctcataatccgcccgccttggcctcccaaagtgctgggattacaggcatgagccatcgtgccaggcctgccatggcgtttgtaaactgtcatggcactggtgggagtgtctgttagcatgctaatgcattataattacagtataattacagcagtgaggacaaccagaggtcactttcattgccatcttggttttgaccggcttctttaccacatgctgttttattggcaaggtctttatgactgtatcttgtgctgacctcctatctcatcccatgacttggaatgcctaacctcctgggaatgcagcccagtaggtctcagccttattttacccagttccctattcaagatggagtcactctggttcaaacgcctctgacactcccaatttttgcaggtgaggaaatggaagccttgaaagattaggtggctcactctaagtaacatcatgtacctggcagggatttctataaagtcataagatgtcagagactatgcttaagaaatatttttactttgaaacactttaagcaaacagttaaaaagtacccaccacactaccctgtaaaaatcttaacattgtgatgcctctgcatcaatttttagaaaaaaacaaagaaaacacaactgaaggccccatgtaccctccccaaatccatcaggtctcctgccttaggaaggcagaatggtgacttgcacacatcgttccaatacatgattttatactcatttcatattatttgaatccacagaaaatagattactgtgcaaaacaataacactttctatatgtccacaaggcttacatgctagacactattctaagcattttacatgcattacttcattgaccacccccccacccacaatcaccctgtgagattgccactactatcccattttacagaaaaagtgaaaaacaagttgaagtaacgtgcccacaggtacacagtatgcttaactttacactaagggtaccttgtatgtagcttcaccaactttctcagcataatttttcatctatctgtgttgagacgtaactctttcatattcactttccaaggaccaaaaacaacccatttatttatccattcttctgctgatgaaatgcaggcttttcccaatcttgctacctaaacaatacttcagtgaagtcttaaaatcattctctgttcacatggcacttctctaggatgcatccaggagtagttgctgggtggttaagtgcacacaaccttccaagattttgcaaattgcctggcacaatatttctcacaatttctactcataaagcagtgtgaattatcgttgttccacgcacttacccacacttgggctttcaaaaatgtgccagctttctgagtgtgagatggtctgtattattttacatttcagtcagtcttggtcagcaggggtggggcagaccacactgaacaggtgacagaaagaccttcaaatacccactccagccatctggctctcctcaaccccaacttcagttcctccaagggagtgggggaaaggtgggaagggttggaaggaaactgaatgttctccaggccaggatgagatgcaagatgagacctggtgctcagggcaatcagaaactgtcaactgaagccaaacagctcagaaccacccacagccgggttcctaaccagcaggtgtgtgtttgtgggtggcttccagtcaacatttcaccccacagccccttaaaaaaaacccaaccctgactcagccaaactaaattcagcttcagattccttaacagaggtaattttgtgcaagatattttctgcatggcaaacagataaataagcacccaaccctggcttccagagtgcttggtctggctatggagatgggcataaccaaaaacacaaacatcacctgacataggaaccaagagaggtggggccacgggtttagaggcacaagggtcagacaaggtcaggccttgaagaatgaagagctgaactggcagagagaggggtgtggcactccaggtgaagggaggcagcacaaggcagaacactctggggggctggcatggggaagggacaggaaagccaaatccaacattgattctgccaaaatctttagtagttagcaccaagtagtcaggcttctactttttttcctttcagctaatctgaattcattaatatttatataattatagtacttatagaactaaaattatttgaaaactcaggttattggacaaataggttcagtataatcccaaatataaacagcttacttcaggataaaataatttctgttcttttggccgggcacagtggctcacacctgtaatcccagcattttgggaggccgaggcgggtggatcacgacgtcaggagatcgagaccatcctggagatcgagaccatcctggagatcgagaccatcctggctaacacagtgaaaccccgtctctactaaaaatataaaaaataacccaggcgtggtggcaggcacttgtagtcccagctactgaggaggctgaggcaggagaatggtgtgagcccaggaggcagagcttgcagtgagcggagatcgcgccactgcactctagcctgggtaacagagtgagactccgtatcaaaaaaaaaaaaaaattcagtttttcacttcattctttgcacattttaaaatttgattagaatgtttagaaataagcacatttcattctataaaaatgacaggtcaggcacagtggctcacgcctgtaatcccagcactttgggaggcagaggtgggtggattgcttgagcccaggagtttgagaccagcatgagcaacatgggaaaaaaaaataaaagttttgtctctacaaaaaaatataaaaaattagctggcagggtggcacacacctgtagccccagctactcgggaggctcagatgggacctgagcctgggaggtcaaggctgcagtaagctgtgatcctgccactgcactccaccctgggcaaccctgtctcaaaaaataaaaaagacagtaaaaatatccctatactggggcaggaactttacaaggtatcctgtggcaaagggagcagagatggggggaaaggggtgctaaaagtttgattggaaagggacttttccatggttacaacaccaactgacatggaagctgcacctctgagagggccctggtcctagaggtcaaccacctgatggagagccttggtaaaccaagccctctttcaccaatctcaggaatcaggtagcacagccaagcactctaacttcacacataaggaaattgatgcagaggttcattgacttgctcaagatcaatcctgccaagaaaaggcacaccatgcctggaacccagatctgatgactccaagacccttcctatgactctggcccccctgcccagccacttctagtgccagttttgggacagtgaagggacatcttcagtgccatgaacagctgctgccgtaggaaggcaagaggatggcagaaccaagatgaccaaaccttcctgaggacaaagctgaacaggcatcagaacaccaacaggagacttctgccccgcccccaccatcctgtgacaccaccacacaatatcagagccttcattttcacctgctcatggcaatccagagcaggtaagattattccatactctactgaaaaagacatcttccaggttggtttcttctcatttcaagaaatgaccagctccatgaacgggcccctatagtcaggacactgctctactattaaaacattttatcctttcattcataatctgacctcttcaataatcagaagcaatgattactcacatgctttagcaatatcactcctttgcctttaagtaattgattcttgctttttgcttcaacacaagtgggtgggccagtgagggagctcctcccagaacaggctgccttttctcctgagagcagcaggcacatgcacttgttccttcgggttgaatctgattgctagcaccagatctcatacatggagaggggtatgtgaagctgagaggggcctgcagtgtgcaggggctagagacatgaacacaacaatggtaagcgtttatatctgctgaggccgaggatcctatagaaaattcagaaacggagtggggaggagtctgatttatgggaactggcagcaaggctaactgcatgagaagcctttcacccttttactgagtccttggatctgtggttaacccttataaaatataattcagattcaaaccacatcactcctcaactcaaaattgtccaaaagctccctgcctccctctgagccagctcaagcccccgtaatgacccatgatgctcatatggccgggcctgtggcctccctggcccctctccttcccttccagctggctccctgcactccatcccaggggcttccttcctgaggacaccagtcaagacccaatctcctctgcctgcaactctccctagagagctacctgctacctccctggcttccttcacgtctttgctcacatttcaccttctcagttgaggccctccctgaccagactatctaaaatcacgactgatctcccaatccagcactccctctgctcttctctgattcactttgtccactacacacatcaccatccagaatactgcgtatcccatttgtttgtcatctgtaaagatccaagatggcaggattttcatctgttctggtccctgctgggtctctggcaaacacaccagcgcctggtgtatgggagtgctcagcacatttctgttaaacagatggaccgctgctgcctatgcaggcctgtgggatggggatggcaacagggtactggtagagatccacacgccaagcgcttgagcccagcatcctgctctcctccacctgccgctgagaccactctaaccccctagcagatatccaaaagccagccaggaaggctgaagccccagccagaactccccagggggcatttgggaaggctaggagttcttgatgctgctgcttttaaagtcaacagaataggcatggccacaggccaaacttgaagacaaatctaggatcccactggcccctttccagcagccatagcccatgatgccacagatattctgtccaaccacaaagggcagtggtctctctcttcagagttgtggaaggagacctgaataggggagccgcaggctatggtgcagaggccactcctaggggccggagtctccagaagggctccaaaggacatggtgctgcacttccccagcgtcacatcctagcaggcaggctggggactccccgagctttcaaatccttgggattctgtcactagcttccaaaacagaaagggctgggccctttatcaaagttactccacaatgcctataattaagggttctctagcaggggactgagaacccacccccactgtcactgtcaggtcccaggctaatctctaatatggtttttcatatgccgagccaggttcgaagaccacctgaaggtctttccacacttgctgcatttgaagggcctctctcgagtatgaaatctcttgtggctaatgagttgtgaactcttgttaaaagttttcccacatatgctgcatttgtggcactttttcccaatgcttatgtcctggagtccagtgagcctggagctctggctgcaagcttctttgcagtcttcgaggggcatctcttcacttggttttagcttctgtaatctcaactttgtgtcctgagaggaagaccgtgcaggcgggctacgttcagcctgtgctgctctggtgtgtttcctctggtgactggaaagggtatgtctcccaatgaactctttcccacaccactgacatttgaaaggtctctctgtagagtggatcctctgatggttaacaaggcgatagtttctatcataagatttcccacatagattacatttatagcgcttctctccactgtgtattcccttatgatctaaaagggttcttttacgtgtaaaggttttcccacattcttgacaccaaaaacgtttctcaccagtgaggatttttggctccacatttggagtcttttcactttcatggcaatcatactgtttttgaagagagtgaatcctctgatgtcggtagagattggaactccatctgaaggctttcccacactccctgcacttatatggcttctctccagtgtgaactctctgatggatgaggaggaatgagtgattgcggaaggccttgccacactggctgcatttgtagggctcctctttggagtgactgctctgaggaacctggaacactgtgtcctgactaaaagatggcccgccctcaggttttcttttcatggcatgcttcttcttatgaacaataaaggctgacctataggcaaagtccttcccacaatcgctacactggtaaggtttctcacctgtgtgaattctctggtggtcaacgagagttttctttctagtaaaagttttcccacactgctgacacagaaatgttttctccacagcgggagcaccctggggctgactgcagtcaggagattgcctgaagccttcacgacattcatcttgtttgtagaatttttcctcctcatgcaacctcatatgacgagtaaagtttgatctccatctaaaggttttcctacatttggtacatttatagggcttctcctgggtgtgaatcctttgatgttcaagaacatatgacttacagtggaaggatttcctgcactggctgcagtcaaagagtttctccccactttggtctcccaaatgatgatcaaaccctgagctgtaggtgagagctgccctatactgattcaattcaagaaatttcttcttagcatgggtttctcggtgcagacggtaggctgacaggcgtcggaaagctttctcacataaatcgcatttataaggcttcactccagtgtgaattttctcatgccgcgcacagttggaactccaccggaaggctttcccacacaccctacatttaaatgctttctcttgagtgtgaagtctctgatgatacgcaagatgggagctatgactgaaagtccttccacagtcactgcacttaaatgacactcccactgtgtgaagactctgcccacgttggtgatgagagctaaggctgaagtcttttccacacacgtcctttttgttccctttcagtccactatgaattctctgatgtaggctgaagcccccaatcatgtgtctgagccccttcccatatttcttgtagtcatagtggtgtgaactcattctgaagtgtttgccacagccatgtttaagggattcctttcttccagaaactctcaaatatgtaacatgttttaagtcaagactattacttcctgatacttcagagtcttttcctgtcctgtgactgaaattggtctcttctttcttaactcttacttgtatgggattttcacattgatccttctgcctgctcttctgttgaaaagattctctgagcccaattccctcagaaacacttgtcgcaggacatcctgatgacacagctaaggtttctgcttcttccaaaggttcctgatttaagatgaatttgtttgttttactctggaggtcatctcctgtaggagcagcaactggattccccttaggctgagctgcctgcatgttcaggccccatggctcccttgcttccaaccaggagatcagagcaggtttggtgaatggtcccaccagggaagccatgttcctataattctccagcatcacatccctgtacaggttcctctgagcagagtccagccacccccactcgtcctgggagaaggtcacctccacatccttgaaagtcatggtctcctggagctgggctgtcagggacctggttggtgttacctggtctcccgggcacccctctctcgggaaaagggcaggcatctgggcagcaggagtatcggattgcccagccaggaagtcacgtgcttctatttcatagggaggctccaggtggtcccccagagcagagctgctcctgagaggtgaagcaagggaccatatctgtgcagatcgcagggctcctgtacccatccaatgcacatctgggctctgggcagggcccgggtccctccaggatgtcccatcaaggtccctctgcagctcctccagcaaggccacagcctcctcgccactctcagggttatgaagctgcacccaaacccggagctccccaggcaggatgctcaggaactgttccagcaccagcagctctaggatctgtgccttggagagaacgtcaggcctcagccaccagcgacagagttcccggagccggctcagagtttctaggggccctgaagactcatggtagcgaagctgtctgaagagctggcggaacagctcctggccagggcggttgagagtctgtggcctggcagcctgcactggagtatagctttcatcctcttcttccttctttactgtctgaagccgccctcgctccctcgaagactgggcctgagctggataggcagcatgccacctgcctggaggcatcactcctgttcagggactaaccagaagagtgcgaaccaagtccaccttagacgtgggtcctcagaagtatcttctcagcagtcaacaatgccaacatttgctgggacatcagaagtcatcagcaagtgactgaaattaccagcatttctgtagtcccagctactcgggaggctgaggcagaagaatcacttgaacccaggaggcggaggctgcagtgagccgagatcatgccattgcactccagccttgcgaaagagcgagactccaccgactcccgccgccgagcgacaatcggtccacccgccgccaccgcagccgcccgtcccgcgcctacctcccggcggctcc

SEQ ID NO: 15209 - RNA, 17836 nt, Homo sapiens
  source 1..17836: mol_type = other RNA
gctgggattacaggcatgagccactgcacgtggctacatgttttgtatttttagtagagacggggtttcaccatgttggccaggctggtctcgaactcctgacctcaagtgatccacctgcctcagcctcccaaagtgctgagattacaggcgttgagccaccatgcccagcccttgaaatttaaatttcaatgtctctaaatgaagttttattggaacacatctacactcatttgtgtgtgtgtgtctgtgtgtgtgtgtgtgtgtgtgtgtgtgtgtgtgtggatggagatagagagagagggatttatgaatttatgataaggaattggcttatagaattaaggaggctggcaagtcccaaatcttcagggtggatgagcaggctggagaaccaggagaatacatattccagtgagagcccagtggcacctgctgtggagcaggattagtagatggtgtgcatgaactctgaaggcagtctgcggaagaattctctcttgcctgagagagagtctggggcagccagactttatgttctcctcaggtcttcaggtgattggatgaagcccacccacagatagagggcaatctgctttcctcaaagtccacaaatttaaacgttaatctcatccaaagcaacctcacagaaacacccagcataatgtttgatcaaatacctggggaccttgtggctcagccaagttgacacctaaaatttaccctcacactccagtcctccaacatcccagcttccctcttacatccctgaatggcagaacccaacaaggaaccagctggcgaagcagcatcgtgcctgttctttgttgcctgtgtttttcattttaagtcggtggagttacaacccatggattcctttgtgtctgcttccttttcattaaaattctgctcatggattcatccctgcagtaggttcattttcaggtggaagtgtaggaagcacaggagatcacagaagacctcagcaggccagctttgcaacatcctaacaaggagacgggaaactgaagtaccacaggaaggagatactctccatctctcaccacccaaagcttcctgggatgctaagggtcatcgttctttttttttttttttcccgctctgttgtccaggctggagtgcagtggcactatctcggctcaccacaacgtccgcctcccaggttcaaacgattctcctgtctcagcctccccagtagctgggatttacaggtgcccgctaccacgcctggctacttttgtatttttagtagagacagggagttcagactggtctcgaactcccgttctcaggtgatctgcccacctcagcctcccaaagtgttgggattacaggtgtgagccaccgtgcctggcctaagcctcactgttcttttcatctttcctgctgagacaggagattgaggatgtggacattttgttgaggaaagaaataggacagacaactcaatgaagtctcagagagccattctaagaacccatgttctatttccagaacccacgtcaggccattactggggggtctgatggggttatgagagaaatgcccagggagggagactggagaaggttcagggaccaagttctggcttctgcccttagaggagccggacctgcagagagagagtgggaaagtggagaaccatcagctcactttccctcacgccatggcaaaagcatctccatcaggcaggactggcttcacaggcaggcagcctgggcagccctgcggggccccacacttagaatggcctccgcctgctatcttgctctgctgtcagggtcttgaaattctgaatggtcttgaacatcatgcactgcacctggcaaaatagccggtcctgatcaggtctcaaggcagccctggactttggaaggcagcactgacgccccactgaggaaaggaatggctgctgaggactgagaactagagctgagactcccaggcagcccctttggaaaacagtttggcatttccccaaaatgttaaatgtggaattatgtgattcagaaaatcacatacaaaattgtctcgtgtcccttttaaacatatagaatgtaactattggaaagagagagaaaaagggcctggcttggtggctcacttctgtaatcccagcactttgggaggctgaggtgggcagatcacttgaggtcaagagttcaagaccaagctggctaacatggtgaaaccctgcctttaccaaaaaaaaaaaaaaaaaaattagccgggcgtggtggcgcacacctgtagtcccaacaggctgaggaagcagcttcacttgtacccaggaggtgcaggttgcagtgagccaagattgcctccactccagctcgagctacagagtgagactctgtctcaaaaaagaaaaaaaaaagagagaaagaagttttggaaacattatttgcccttagccatgttgtgggtttatttcctacactgagtcatattatgtgtcttccaacatgtctggagcagttgctactccctgtacaccaggtccagtgactataatgtcatcaatataatggaccagtgtgtcgtcctgagggtgaaaaggttctcaaaggacctgggaactagatcatgagctgggcggcagagttgaggcagccttgagatagggtggtgaaggtgtatctagctgaaagcaaactgttcctgatggtctttactcacaggtatagagaaacattcaccagatgggtaactgggcagccaaggggataatcggatcgggtgtgccacacttcgcctgccccgcttgcttttggttgcttgctctttgttattttttcccccatgaagctgaaggccacgatagctgaaggctatgctattgaacactgtaactcaacttttacgtgctaccttatagataacatttataagtcaccataacaaccacttatttttcaggaacttggggcagatcctgtccagttcaaaccagttgagactgccaacccttcaactgggcctgtacacatgcccaagaggtggccttttgacatcagagggccaaaaactccaccctcagatcatgttaacgccaccattttctgcacatatgtcatatgaaccccaattatgactgcatttttccccactgccaatcacctttccccatgcctcagaccaccctacttctctaacctataaatctctctaagcctcatctttggggaggtgaatttgagagccattctcccatctcctcactggacagccttgtgaataattcttctctcttttgcaaaacccatgtcacagtgattgatttactgtgtgagaacagaacaaacctgggcctggctcagtaacaactgcaaaccagttgtcagacgtatcgtttgctcagcactgaaaccacatgtggaaacagcacctgcacttggaatcactagttaattaagtttacaattaatccaattgtcattctccaagatccatctgtcttctgcacaggctgagtaggtgagctaagtggagatgtgttcccgtctttgatggtggcactaatctcaacaatctctccaggaatgtggtattagtttgctttaatatttttgtgaatgaggcagctctagtggcttctacttggccttttctaccagaattacttttactgtatggatcagggaactagtgtgggattctgcccattgttgactatgtctattctaattacgcattctagaaccagggaaataaccataggatgggttcaggaatctactagatctactgtgagatgaatctgagccaaaaagcccattgatcacctgacctccatacactcttactctgaggaaccatggtggcattttgagtctcctgtaattactgctagttcagaactagaggctggttatcccagaaaagtctaattatttgcccttcccaatgcacaatcactctgataaatggccttgggtgcctttggggaggcctaggaagataaaaagtataaattattgtcagtgcagcagggtcctacttcaaagggacctggcctatcctttattcaagaagctgtgggtttgtgaactagatcaagacttggaattgactgagtgattgtaactctgtgttggtaatttaggtcagactttattcaccagatctggagctttcctacttactcggatcaagtaaaactttagtaggcagcccatccatttcagttctcaggacactatgatcagcaggcagacatcacagatctctgtgggtcagaccattcaggatcctgctttggctgcactgtccatggcagtcaccacaccaattgtgtttttggtgactaagtgttaccatatggtccctgcctcctcaggattccatcagccccactgcacttcagggagcatttcccactgtaatgtggcctgtatagaatatctggcactctctacatgaatttatttctcataatgaagtgtcctctggaccctccctgggtgggtgagcaggtatttacatgataaatactcaagcatttttatctccttaagcatttacatatcttcctctacagtataccaacgaagttctcgcatttcaactcattcagtgcaggttatgtttgcattcgtgttttttttttcttttggagatgagttctcactatattgcccaagccagtctcaaactcctggcctcaagcaatcctcccacctcagcctcccaagctgggattacagtgagtccatatctcaacaactcaaagcaaatgaagacagccattctcagcttctcaagttaaaacaatgaaccacaaatctctgcttaattatcccatatcgaataattcagcttgatctgactttatattccttccacgatgatcctgcacccttgttaccgcaaaaggttcccaatccagaccccaagagagggttcttggatctcgcacaagaaagaattcagggcgagtccgtaaagagaaagcaagtttattaagtaaaggaataaaagaatggctactccatagacagagcagccccgagggctgctggttgtctattttatggtttcttgatgatatgctaaacaaggggtggattattcatgcctcccctctccaggccatatagggtaacttcctgatgttgccatggcaactgtaaactgtcatggcactggtgggagggtagcagtgaggatgaccagaggtcattctcatcaccgtcttggttttggtgggttttagctggcttctttactgcaacctgctttatcagcaaggtctttgtggcctggatcttgtgccaatctcctatctcatcccgtgacttagaatgccttaaccgtctgggaatgcagcccagtaggtctcagcctcattttgttacaggaaaggggtcccgatccagactcttaagagagttcttggatctcgtgcaagaaaggattcagggcaagtccgcagtgcaaagcaaaaacaagtttattaagaaagtaaagtggtgaaaggacagctactccatagagtaggatggagtaacctctaacctgaggtcagtcaagtgtccttgccttttattaagaggggcctctaactcactctgtcttaggagaaactccaactcccctaagttgggcctctaacccaatcccatttgttactcgggtaccccatcacttacccaaagtcgtccaatcagtgctgcagtctatttctttggggttggggggatttcttcagtatcatcctttctgtggtttgccagaaatatgttacaggaccccaacacttacgcaaaggtagccgttgggtcaacgtttctgcactatagtcccttctgtggtcaccagaaatatgttacaggaaaggggtcccaattcaatcctagagggtaggaatgcctaactttctgagaatgcaggccagtaagtctcagcctcattttcccagccctcactcaaaatggagtcgctctggttcaaatacctctgacacttttacccagcccctattcaacatggagttgctctcgttccaatgcttctgacgctatctctacagattccccaggtttctataaaaattggcaaaattatgcaatttggagagtactgtatctcctcagtcacattttgcacttcacttttttttttttttaattgagacaaagtttcactctgtcgcccaggctggagtgcagttgtgcgatctcggctcactgcaacttccacctcctgggttcaagtgattctcctgcctcagcctccccagtagctaggattacaggcacacaccaccacacccggctaatttttgtatttttaatagagatggggtttcaccatattggccaggctggctggtctcaatctcctgatctcgtgatctgcccgcctcagcctcccgagtagctgggactacaggcgcccgctgccacgcccggttaattttttgtatttttactagagacggggtttcaccgcgttagccagcatggtctcgatctcttgacctcgtgatctgcccgcctcagcctcccaaagtgctgggattacaggtgtgagccaccgtgcctggccaaaaaaataatttttttaaaaggactccaggcaatgatagactggattaagaaaatgtggcacacatacaccatggaatactatgcagccataaaaaatgatgagttcatgtcctttgtagggacatggatgaaggtggaaataatcattctcagtaaactatcgcaagaacaaaaaaccaaacaccgcatattctcactcataggtgggaattgaacaatgagaaaacatggacacaggaaggggaacatcacactctggggactgttgtggggtggggggagggggggagggatagcattgggagatatacctaatgctagatgatgagttagtgggtgcagcgcaccagcatggcacatgtatacatatgtaactaacctgcacattgtgcacatgtaccctaaaagtataaaaaaaaaaaaaacaaggactccaggcatggtggctcacacctgtaatcccagcactttggcaagctgaggcaggtgggtcacttgaggtcaggagttcaagaccagcttgggcaacatggccaaaccttgtctctacaaaaatacaaaaattagctgggtgtggtggtgcacgcttgtagtcccagctagtcaggaggctgaggctggagaatcgcttgagcctgggaaagtggaggttgcagtgagctgagatcgtgccactgcactccagcctgggtgacagggtgagaccttgtctcaaaaaaaaaaaaaaaaaaaaagcaaaacgcaaaaagcagtggtgaccataggtcatgagcaacgtcagcggacttttggaagacatatacctcagggaaggccattacatgttcttcaggcaaaaggtggttaactaacactcaaagtctcattgtgaccctcccttctgctccctgccccagcattagtagctgggacctctccacagaagcacagatccaaaggccacagggcccctccctgagcacagacactatgtcagcccagcagtccactcctccaccataggtctgagttcagctccacaaggtccctcttccaatctcccacctttcaacaattctagccacgtctctttgttcctgctttgcactttgctccacatgaggtgggatcaataaactaccatcactcaaaactggttcggatgttgaaactgatgacactgcagacaccaagaggttatgaaaaagtttactactcacatgaggccttctagggaaagcaaagcgggcacccacgccagtctgttgggcttcagtgaaaggacgaacaagtggctctggtttttgttgtggttatgagagctcagtgcatttgacagtcagggtttgcacagtttgaacttcccctctgacgcaaagaggaagtggctgggctttcttatcagcttgtccagatccaggcaaactgagggggagagcttgaatgctattagcagacaaacgtcaaacatggggagactctattctagctcccccagtcctggggtggcagctgcttagcagttgctacctccaagacaccttggcattttcttcttgcctttttagctacttaaatatagtacacttctttataaggtctttgctaaaataactggtgtggtttctggcaactaaaacctggctgatataaaatctccttgctgttcttagcagggttaacattaactttaaaaggtgtggtagctggcatacaagtatttactctccttttcctcatctaataaagtagaatgaaaaacatctccatcttctggatcccatttcttcattaaaattatgagtttacagcttctggcttcacttgttatttattaagcaaaattaaggagatttaggcaaggaggagcttataatttcctataaagtgcatgtcttggtgactgtgcgtcagtatatagagaacatcctcatttttaaaaaaactgtggcctggtatttcatcatagatgtactagagttacttaagcgttcgtttactaatagccatttgtattgctcctgttaccagaaagcggtcgtgatccagtccccaagagagagttcttggaccttgctcaagaaaagaattcgggcgagtccacaaagtgaaagtagttaatattaagaaagtaaagaaatacagaatggctactccataggaagagtagccccaagggctgctggttgcctatttttatggttatttattgattatatgctaaacaaggggtagattattcataagtttcccgggaaaggtgtgagcaattaccagaactgagggttcctctcctttttagaccatatagtgttacttcctgatgttgccatggcattttttttttttttttttgagacagagtcttgctctgtcacccaggctggagtgcagtggcaccatcttggctcactgcaacctccaactcccgggatctagagattctcctgcctcagcctctcaagtagctgggattacaggcacgtgccaccatgcccagctaatttttgtattttttagtagagacagggtttcaccatgttggccaggctggtctcaatctcctgacctcataatccgcccgccttggcctcccaaagtgctgggattacaggcatgagccatcgtgccaggcctgccatggcgtttgtaaactgtcatggcactggtgggagtgtctgttagcatgctaatgcattataattacagtataattacagcagtgaggacaaccagaggtcactttcattgccatcttggttttgaccggcttctttaccacatgctgttttattggcaaggtctttatgactgtatcttgtgctgacctcctatctcatcccatgacttggaatgcctaacctcctgggaatgcagcccagtaggtctcagccttattttacccagttccctattcaagatggagtcactctggttcaaacgcctctgacactcccaatttttgcaggtgaggaaatggaagccttgaaagattaggtggctcactctaagtaacatcatgtacctggcagggatttctataaagtcataagatgtcagagactatgcttaagaaatatttttactttgaaacactttaagcaaacagttaaaaagtacccaccacactaccctgtaaaaatcttaacattgtgatgcctctgcatcaatttttagaaaaaaacaaagaaaacacaactgaaggccccatgtaccctccccaaatccatcaggtctcctgccttaggaaggcagaatggtgacttgcacacatcgttccaatacatgattttatactcatttcatattatttgaatccacagaaaatagattactgtgcaaaacaataacactttctatatgtccacaaggcttacatgctagacactattctaagcattttacatgcattacttcattgaccacccccccacccacaatcaccctgtgagattgccactactatcccattttacagaaaaagtgaaaaacaagttgaagtaacgtgcccacaggtacacagtatgcttaactttacactaagggtaccttgtatgtagcttcaccaactttctcagcataatttttcatctatctgtgttgagacgtaactctttcatattcactttccaaggaccaaaaacaacccatttatttatccattcttctgctgatgaaatgcaggcttttcccaatcttgctacctaaacaatacttcagtgaagtcttaaaatcattctctgttcacatggcacttctctaggatgcatccaggagtagttgctgggtggttaagtgcacacaaccttccaagattttgcaaattgcctggcacaatatttctcacaatttctactcataaagcagtgtgaattatcgttgttccacgcacttacccacacttgggctttcaaaaatgtgccagctttctgagtgtgagatggtctgtattattttacatttcagtcagtcttggtcagcaggggtggggcagaccacactgaacaggtgacagaaagaccttcaaatacccactccagccatctggctctcctcaaccccaacttcagttcctccaagggagtgggggaaaggtgggaagggttggaaggaaactgaatgttctccaggccaggatgagatgcaagatgagacctggtgctcagggcaatcagaaactgtcaactgaagccaaacagctcagaaccacccacagccgggttcctaaccagcaggtgtgtgtttgtgggtggcttccagtcaacatttcaccccacagccccttaaaaaaaacccaaccctgactcagccaaactaaattcagcttcagattccttaacagaggtaattttgtgcaagatattttctgcatggcaaacagataaataagcacccaaccctggcttccagagtgcttggtctggctatggagatgggcataaccaaaaacacaaacatcacctgacataggaaccaagagaggtggggccacgggtttagaggcacaagggtcagacaaggtcaggccttgaagaatgaagagctgaactggcagagagaggggtgtggcactccaggtgaagggaggcagcacaaggcagaacactctggggggctggcatggggaagggacaggaaagccaaatccaacattgattctgccaaaatctttagtagttagcaccaagtagtcaggcttctactttttttcctttcagctaatctgaattcattaatatttatataattatagtacttatagaactaaaattatttgaaaactcaggttattggacaaataggttcagtataatcccaaatataaacagcttacttcaggataaaataatttctgttcttttggccgggcacagtggctcacacctgtaatcccagcattttgggaggccgaggcgggtggatcacgacgtcaggagatcgagaccatcctggagatcgagaccatcctggagatcgagaccatcctggctaacacagtgaaaccccgtctctactaaaaatataaaaaataacccaggcgtggtggcaggcacttgtagtcccagctactgaggaggctgaggcaggagaatggtgtgagcccaggaggcagagcttgcagtgagcggagatcgcgccactgcactctagcctgggtaacagagtgagactccgtatcaaaaaaaaaaaaaaattcagtttttcacttcattctttgcacattttaaaatttgattagaatgtttagaaataagcacatttcattctataaaaatgacaggtcaggcacagtggctcacgcctgtaatcccagcactttgggaggcagaggtgggtggattgcttgagcccaggagtttgagaccagcatgagcaacatgggaaaaaaaaataaaagttttgtctctacaaaaaaatataaaaaattagctggcagggtggcacacacctgtagccccagctactcgggaggctcagatgggacctgagcctgggaggtcaaggctgcagtaagctgtgatcctgccactgcactccaccctgggcaaccctgtctcaaaaaataaaaaagacagtaaaaatatccctatactggggcaggaactttacaaggtatcctgtggcaaagggagcagagatggggggaaaggggtgctaaaagtttgattggaaagggacttttccatggttacaacaccaactgacatggaagctgcacctctgagagggccctggtcctagaggtcaaccacctgatggagagccttggtaaaccaagccctctttcaccaatctcaggaatcaggtagcacagccaagcactctaacttcacacataaggaaattgatgcagaggttcattgacttgctcaagatcaatcctgccaagaaaaggcacaccatgcctggaacccagatctgatgactccaagacccttcctatgactctggcccccctgcccagccacttctagtgccagttttgggacagtgaagggacatcttcagtgccatgaacagctgctgccgtaggaaggcaagaggatggcagaaccaagatgaccaaaccttcctgaggacaaagctgaacaggcatcagaacaccaacaggagacttctgccccgcccccaccatcctgtgacaccaccacacaatatcagagccttcattttcacctgctcatggcaatccagagcaggtaagattattccatactctactgaaaaagacatcttccaggttggtttcttctcatttcaagaaatgaccagctccatgaacgggcccctatagtcaggacactgctctactattaaaacattttatcctttcattcataatctgacctcttcaataatcagaagcaatgattactcacatgctttagcaatatcactcctttgcctttaagtaattgattcttgctttttgcttcaacacaagtgggtgggccagtgagggagctcctcccagaacaggctgccttttctcctgagagcagcaggcacatgcacttgttccttcgggttgaatctgattgctagcaccagatctcatacatggagaggggtatgtgaagctgagaggggcctgcagtgtgcaggggctagagacatgaacacaacaatggtaagcgtttatatctgctgaggccgaggatcctatagaaaattcagaaacggagtggggaggagtctgatttatgggaactggcagcaaggctaactgcatgagaagcctttcacccttttactgagtccttggatctgtggttaacccttataaaatataattcagattcaaaccacatcactcctcaactcaaaattgtccaaaagctccctgcctccctctgagccagctcaagcccccgtaatgacccatgatgctcatatggccgggcctgtggcctccctggcccctctccttcccttccagctggctccctgcactccatcccaggggcttccttcctgaggacaccagtcaagacccaatctcctctgcctgcaactctccctagagagctacctgctacctccctggcttccttcacgtctttgctcacatttcaccttctcagttgaggccctccctgaccagactatctaaaatcacgactgatctcccaatccagcactccctctgctcttctctgattcactttgtccactacacacatcaccatccagaatactgcgtatcccatttgtttgtcatctgtaaagatccaagatggcaggattttcatctgttctggtccctgctgggtctctggcaaacacaccagcgcctggtgtatgggagtgctcagcacatttctgttaaacagatggaccgctgctgcctatgcaggcctgtgggatggggatggcaacagggtactggtagagatccacacgccaagcgcttgagcccagcatcctgctctcctccacctgccgctgagaccactctaaccccctagcagatatccaaaagccagccaggaaggctgaagccccagccagaactccccagggggcatttgggaaggctaggagttcttgatgctgctgcttttaaagtcaacagaataggcatggccacaggccaaacttgaagacaaatctaggatcccactggcccctttccagcagccatagcccatgatgccacagatattctgtccaaccacaaagggcagtggtctctctcttcagagttgtggaaggagacctgaataggggagccgcaggctatggtgcagaggccactcctaggggccggagtctccagaagggctccaaaggacatggtgctgcacttccccagcgtcacatcctagcaggcaggctggggactccccgagctttcaaatccttgggattctgtcactagcttccaaaacagaaagggctgggccctttatcaaagttactccacaatgcctataattaagggttctctagcaggggactgagaacccacccccactgtcactgtcaggtcccaggctaatctctaatatggtttttcatatgccgagccaggttcgaagaccacctgaaggtctttccacacttgctgcatttgaagggcctctctcgagtatgaaatctcttgtggctaatgagttgtgaactcttgttaaaagttttcccacatatgctgcatttgtggcactttttcccaatgcttatgtcctggagtccagtgagcctggagctctggctgcaagcttctttgcagtcttcgaggggcatctcttcacttggttttagcttctgtaatctcaactttgtgtcctgagaggaagaccgtgcaggcgggctacgttcagcctgtgctgctctggtgtgtttcctctggtgactggaaagggtatgtctcccaatgaactctttcccacaccactgacatttgaaaggtctctctgtagagtggatcctctgatggttaacaaggcgatagtttctatcataagatttcccacatagattacatttatagcgcttctctccactgtgtattcccttatgatctaaaagggttcttttacgtgtaaaggttttcccacattcttgacaccaaaaacgtttctcaccagtgaggatttttggctccacatttggagtcttttcactttcatggcaatcatactgtttttgaagagagtgaatcctctgatgtcggtagagattggaactccatctgaaggctttcccacactccctgcacttatatggcttctctccagtgtgaactctctgatggatgaggaggaatgagtgattgcggaaggccttgccacactggctgcatttgtagggctcctctttggagtgactgctctgaggaacctggaacactgtgtcctgactaaaagatggcccgccctcaggttttcttttcatggcatgcttcttcttatgaacaataaaggctgacctataggcaaagtccttcccacaatcgctacactggtaaggtttctcacctgtgtgaattctctggtggtcaacgagagttttctttctagtaaaagttttcccacactgctgacacagaaatgttttctccacagcgggagcaccctggggctgactgcagtcaggagattgcctgaagccttcacgacattcatcttgtttgtagaatttttcctcctcatgcaacctcatatgacgagtaaagtttgatctccatctaaaggttttcctacatttggtacatttatagggcttctcctgggtgtgaatcctttgatgttcaagaacatatgacttacagtggaaggatttcctgcactggctgcagtcaaagagtttctccccactttggtctcccaaatgatgatcaaaccctgagctgtaggtgagagctgccctatactgattcaattcaagaaatttcttcttagcatgggtttctcggtgcagacggtaggctgacaggcgtcggaaagctttctcacataaatcgcatttataaggcttcactccagtgtgaattttctcatgccgcgcacagttggaactccaccggaaggctttcccacacaccctacatttaaatgctttctcttgagtgtgaagtctctgatgatacgcaagatgggagctatgactgaaagtccttccacagtcactgcacttaaatgacactcccactgtgtgaagactctgcccacgttggtgatgagagctaaggctgaagtcttttccacacacgtcctttttgttccctttcagtccactatgaattctctgatgtaggctgaagcccccaatcatgtgtctgagccccttcccatatttcttgtagtcatagtggtgtgaactcattctgaagtgtttgccacagccatgtttaagggattcctttcttccagaaactctcaaatatgtaacatgttttaagtcaagactattacttcctgatacttcagagtcttttcctgtcctgtgactgaaattggtctcttctttcttaactcttacttgtatgggattttcacattgatccttctgcctgctcttctgttgaaaagattctctgagcccaattccctcagaaacacttgtcgcaggacatcctgatgacacagctaaggtttctgcttcttccaaaggttcctgatttaagatgaatttgtttgttttactctggaggtcatctcctgtaggagcagcaactggattccccttaggctgagctgcctgcatgttcaggccccatggctcccttgcttccaaccaggagatcagagcaggtttggtgaatggtcccaccagggaagccatgttcctataattctccagcatcacatccctgtacaggttcctctgagcagagtccagccacccccactcgtcctgggagaaggtcacctccacatccttgaaagtcatggtctcctggtctcccgggcacccctctctcgggaaaagggcaggcatctgggcagcaggagtatcggattgcccagccaggaagtcacgtgcttctatttcatagggaggctccaggtggtcccccagagcagagctgctcctgagaggtgaagcaagggaccatatctgtgcagatcgcagggctcctgtacccatccaatgcacatctgggctctgggcagggcccgggtccctccaggatgtcccatcaaggtccctctgcagctcctccagcaaggccacagcctcctcgccactctcagggttatgaagctgcacccaaacccggagctccccaggcaggatgctcaggaactgttccagcaccagcagctctaggatctgtgccttggagagaacgtcaggcctcagccaccagcgacagagttcccggagccggctcagagtttctaggggccctgaagactcatggtagcgaagctgtctgaagagctggcggaacagctcctggccagggcggttgagagtctgtggcctggcagcctgcactggagtatagctttcatcctcttcttccttctttactgtctgaagccgccctcgctccctcgaagactgggcctgagctggataggcagcatgccacctgcctggaggcatcactcctgttcagggactaaccagaagagtgcgaaccaagtccaccttagacgtgggtcctcagaagtatcttctcagcagtcaacaatgccaacatttgctgggacatcagaagtcatcagcaagtgactgaaattaccagcatttcgactcccgccgccgagcgacaatcggtccacccgccgccaccgcagccgcccgtcccgcgcctacctcccggcggctcc

SEQ ID NO: 15210 - RNA, 4084 nt, Homo sapiens
  source 1..4084: mol_type = other RNA
gctgggattacaggcatgagccactgcactcagccccatttgctcttccaaaattctggtttctccaagacagggtcttgctctgttgcccaggctggagtgcagtggtgcaatcacggctcactgcaacctccctctcctaggctcaaacaatcctcccaactcaccctcccaattagctgggacacagatacataccaccagtctggctttttatttttttgtagatccggtgtctcactatgttgcccaggctagtctcgaactcctggacctaagtgatcctcccacctctgcctcccaaagtgctgaggttacaggtgtgagtcaccacacccggccgaagagaacattttactcatagtagaggctaaagactatgataaaataagcatttacagagaatggagactcatcctgtgaggccttaatttttctctatgttcaaggcagttaattgctcagagtatgggtttggaggatctgtaccacaaacttaaaagtaccaagctaacaaatcactcattttgaaagtctactacaaattcataggccatctacccaaatggattttctcctatcaactctagctgcagagcaacatggtgattcagaataggtgcctggataggaagaggcataccgtgaatctaaggactgtattgaatagtaaggctaacaagagtcaggcatctgcaggtgctgatgaactagagacaggaagggaccgagttaacatttcaggtggccaaggctctccttggaagctgtaaaccaagactgaaggctaatttactctctctgtcctgcaaatctgctttgatatggagcaatacccatggatgcttaagtagctagctactatatcggctttttttttttttgtccctcaattaaatgccttaagacctgacattccaagagaaaacaaaaaccatactttggtttctaaggatgtatgactgggtcccggccttcagaggatggcagacagatgggaacacaagtataagtagactagagtatcccataattgtcaactctggcaaggtaaagatgaagctgcttatgtggacaactcgtggggtacctaagtaaatctgggagccaggtacgtgcaaagtggtcagtggtagaagccctcatgaaggcaggaatgctgcaaacctccacttactgccttccaggaccacttaagtcatagtggtaagagctgctagaagtagtcgttaccaacttgattaccagcaatacacaatgatgtcaagaagacattccacatccttctgtcatcactagctctcatttcaaccactaaaataggtaacagctatagacaaaaaaaaagggagacatgaaacattcatggctgttcaagttagaaaactatggcagcggctatattaacaaaaatacaaacgtgtacactaattacaacatttatctacagtcattttaccagttgtgcagcctaaactgccattatcttgtttagtcattcctaagatgcgttatttctgacatcgaaatatcctgaaattgggaaactattgacccaaccccaactgtgttagaactgcatgaacacctaagatgaaggaccagcatcacagcagcacatcaggccaacaaaggcagaagtccagcagcaggagagggcaatcgcacgaggacagcatcgtgaggtcagctcaccgacactctaggtgtgcaggcttatcctgatgacaagagccatggacctcaccatgtgtctgaaaaccgcaatgttgctacttaaatgctaagcctttaatggtgcattaatagatggttaagtagcatattagcagcttaaatctacataagtcagctgtgtactgactgtacctcacagtaacaaattcaccaaatctgtatcttttcttctttgtaacaatgttaaatattggtatatctcagttctcaggtgtgattccagcagctatggtgagacccattgctgctcctgaatctccactttcatttgccttcactggtgtcactgtcgctgtcactgctgctgtcagtatcactgtcactggtcaatgcagttagattacttagggcttccttttgttcctggttgattgcaaaatcactcattactctctgggtgaggccctcacaaataggtaagctgaaggcacttgccagctctactacttcaatggcctgggaagggctgttagacacttttgcactgtccataagctcattcagcaactcacttctaggaatcttattatgcttcctgaaaagccccaacattttccaggcttcctgagttctcccagcccttaaaaagaggatagctatacagttgagagaggtggctggccaatcctgagcagtctgtctgatgggttggctttcatacgcagatttgatatcagcagcacagtcagcaaatgccacctgaagctctggtgggtgcttgtcccttgccatgagcatcaggatctcttctctcaggtcactgcggaaagtatgaccatattctttactatctttccaaattttaggaatcacttctagccgattggccacatccaatgcttggagaagatgtatcattgtttgggagtggggaaagtaggctgaaggtatcaggtcctcataccacttcaaggtaacatcaatttgttccattagacaaatcaaatcgaagaacttggaataatagaaattacgatgttgatcaggtccaatgaatttccagttgtctccggtttttaaaaggccatgtacttggtaggcaagttctagatctctgagagatgagcatatgctcatggctgactgaaaaaacttatcatcatccgggtcctttggagaaaatctctttcccattaattcattcattatatcataaatgatgaaggatgatctctttaaagggtctccaggttgatcaaacaggcgaataatatggtgatatgttgcaagcgagggttctattccaatggctttcatttcacgtaaaacctgtaaggctggcgatcttgcaaacacatgaaatcttcggagacatttcagaatggtattaaaagtctgaagatttggtttcaccttctgtgcaaccatgtgtcttagcagctccagtattttactccatttttcctcaaatttctcatttatcgcacatactgttgcttcaatcaatgcattaaatgtgtatacatcagcatggagtctgttgtttagtaactcagtgtacaagtttaatgcctgctcataagctcggtgcttcaccattcctcggatcattgtgcaataggaatgttcatttttctctggcattagagaaaagattctctcagcgttgttttttgctcgccatgtaactccaaactgatgaccagctttcctcctagatgtctcatcattttcctcttccaatgcttctgactgtccagtttgttgaaaatggtaatcagttgagggctcctggtcaccatagtaacacaataaatccaagagactatttgttgtttcaagagacacagtggttcctgcttgcaaaagctgatcaaacatgtccacagaggctttgacttttctgagctcaattcgttccttcagggcggcttcacttatgtctttgatctgaggttcaaagtactcaggcattaaacacggtatatgaggttcagctatgtccttctgaaaatatttggggtatgaattaataataaacttggccacattctccccggatttctttgccagtaaaaatgaacgagattccaaagatgatgctggcataaggtaaggatcatcttgaaacacataaggcacagctgtggtatccctgtttactgtggatgcaagtgcctgaagaacggctactttatcccaagttttcttttttggaattactacttcttcaatccctgttacatcagttccttcaacctttgagagggttgcactaccagaataaaatctgcagctgcgtgcctgttcacacaaacccgcccgccgacccgtcagcggctggccaagcctgctgcggaggcccagccagcgaacagcagatacaaccgccatctttgatttctct

SEQ ID NO: 15211 - RNA, 2248 nt, Homo sapiens
  source 1..2248: mol_type = other RNA
gctgggattacaggcatgagccactgcacttcgccccctgcctcttctaagaagcttccgccgcttaatccctccattggcttcccactgcctggagcatctggctaactcttgcccttgtctggagggtagctgaagcacagctcccattttctcagctttcacacacgcaaggccatgtgtcctctgctctggccctctgcctgtctgcccagggcagagcccagcacgaggctggcccagctggatatgcatggagcatacctgggttgcattaaagtgctccccacttctgcttgccaagttcccactcagccctcaacatctggctcagatgctccctcctcagagagctctttcctgactccttggactgggtcatgggcactgtctgtgtaccccctccccccagccatgcttccctctgtcacaaccctgatgttgctgtgccagtctgtacttccagcagttgggagcccgtatggaccagggctaggactggttcttctagggccccagaaccaacacaggcctgagcacaaggtgtcagtaaaggctttctaaataaatggaatatcactcctctccagagagctcataatcatccctcaaaacccagctcaaatgccccttcccagaagctctcacctccccctctcatcttccctcacccgcttcattggtgactcaaagcatggagcataccccttgatgacagtacacgtcacactgtatttttgtgagcaccttaatgtggtttccccagctctccatggctgactgggacctctcaagagccaggcccaggtctgtccatctccatgcccacagggtctgggccagagaaggggctgaagaaatagtttttggtgagcttctgggtcctgtgagggatcttaactccatgcccagctgagctgaactctaattctccgcatggtttggggttggtggggctcctggtgccccggacacaatggcaaatatgaaggctgcccaggacctggaggactcagcgaccctgcctctgccatttggctgtgagtttctgtaggagctcatgtggtcgccggcggaacttcttctgggtgaagtagaagaggatggggtccagcacgctgttggcactggcaaacggccgcgtgcctttgtaggccgctgcaaaggcctccaatacagtgcaggggacgcccggcgtcgagcgcactgccaggtaggctgtcttggtgatgtgaaaaggcaggaagctgatggcaaaggcagcagccaccaccacggccatgcgggccgccttgccacgccgctcctgggccacaggctctgccgggccatcctggcggcacaggcggcaggccaggagacagtagcaggccagcagggcagcaaagggcagcaggaagccgatgacagtgagagccatgccatagggcatatagtgggtggccagggcaggcgggctgaggtcatagcagacagtgcggttacgctggatgcctgtggcagcgaagatggctgtgggcaggcactgggttgtcacggccagccacacggctacacacactagccaggcagcccggcggcccccacgtttgtgccagggggccagcgggtggcagatgcccaggtagcgctggaagctgatgcaggtgaggaagaggatgctgccgtgcaggttggcatagaagaggaagcggaccaggcggcaggcgaagtcgccaaagggccagtgatcaccttgggcatagttgtagatgagcaggggcagggagcaggcatatagcaggtcagccagagcaaggtttagggtgtacacggccgtgcgggtcagggcccggcgggacgtgcagatctgggtaatgacacagatgttcagcggcaggccagccgccagcaccgccgaatacacaggtggcagcagcagttgcttgaagttctcgcggtagacacaggtggtgggtggcaagcccagagcctggcctgtgccattgtcccattccatggctgcccaggtgggtttcctatgttcagggaggcaggggctcactgaggaccgcacccatctcctcagcctgaactccgccttccaaagccatggttcttctggcagaggtcttgttatccaagagttagcaagtgcctcgcttgcagtccgtgaagtgctggagcaaattcccactcgtggagcagcccctgctgccagtcagttctgtgcctgaaactgtcgcgtgcaatgttctggcagaagtct

SEQ ID NO: 15212 - RNA, 2390 nt, Homo sapiens
  source 1..2390: mol_type = other RNA
gctgggattacaggcatgagccactgcacttcgccccctgcctcttctaagaagcttccgccgcttaatccctccattggcttcccactgcctggagcatctggctaactcttgcccttgtctggagggtagctgaagcacagctcccattttctcagctttcacacacgcaaggccatgtgtcctctgctctggccctctgcctgtctgcccagggcagagcccagcacgaggctggcccagctggatatgcatggagcatacctgggttgcattaaagtgctccccacttctgcttgccaagttcccactcagccctcaacatctggctcagatgctccctcctcagagagctctttcctgactccttggactgggtcatgggcactgtctgtgtaccccctccccccagccatgcttccctctgtcacaaccctgatgttgctgtgccagtctgtacttccagcagttgggagcccgtatggaccagggctaggactggttcttctagggccccagaaccaacacaggcctgagcacaaggtgtcagtaaaggctttctaaataaatggaatatcactcctctccagagagctcataatcatccctcaaaacccagctcaaatgccccttcccagaagctctcacctccccctctcatcttccctcacccgcttcattggtgactcaaagcatggagcataccccttgatgacagtacacgtcacactgtatttttgtgagcaccttaatgtggtttccccagctctccatggctgactgggacctctcaagagccaggcccaggtctgtccatctccatgcccacagggtctgggccagagaaggggctgaagaaatagtttttggtgagcttctgggtcctgtgagggatcttaactccatgcccagctgagctgaactctaattctccgcatggtttggggttggtggggctcctggtgccccggacacaatggcaaatatgaaggctgcccaggacctggaggactcagcgaccctgcctctgccatttggctgtgagtttctgtaggagctcatgtggtcgccggcggaacttcttctgggtgaagtagaagaggatggggtccagcacgctgttggcactggcaaacggccgcgtgcctttgtaggccgctgcaaaggcctccaatacagtgcaggggacgcccggcgtcgagcgcactgccaggtaggctgtcttggtgatgtgaaaaggcaggaagctgatggcaaaggcagcagccaccaccacggccatgcgggccgccttgccacgccgctcctgggccacaggctctgccgggccatcctggcggcacaggcggcaggccaggagacagtagcaggccagcagggcagcaaagggcagcaggaagccgatgacagtgagagccatgccatagggcatatagtgggtggccagggcaggcgggctgaggtcatagcagacagtgcggttacgctggatgcctgtggcagcgaagatggctgtgggcaggcactgggttgtcacggccagccacacggctacacacactagccaggcagcccggcggcccccacgtttgtgccagggggccagcgggtggcagatgcccaggtagcgctggaagctgatgcaggtgaggaagaggatgctgccgtgcaggttggcatagaagaggaagcggaccaggcggcaggcgaagtcgccaaagggccagtgatcaccttgggcatagttgtagatgagcaggggcagggagcaggcatatagcaggtcagccagagcaaggtttagggtgtacacggccgtgcgggtcagggcccggcgggacgtgcagatctgggtaatgacacagatgttcagcggcaggccagccgccagcaccgccgaatacacaggtggcagcagcagttgcttgaagttctcgcggtagacacaggtggtgggtggcaagcccagagcctggcctgtgccattgtcccattccatggctgcccaggtgggtttcctatgttcagggaggcaggggctcactgaggaccgcacccatctcctcagcctgaactccgccttccaaagccatggttcttctggcagaggtcttgttatccaagagttagcaagtgcctcgcttgcagtccgtgaagtgctggagcaaattcccactcgtggagcagcccctgctgccagtcagttctgtgcctgaaactgtcgcgtgcaatgttctggcagaagtctgcgccgcgcagcaccagctggtccggcccagatgtcactcgcccaggcgctgctaggaggcgaacccgtcaaatgaggggaccgtgtagacggcggcagcagctccggccccagcgtccctggaacccagaggagccagagc

SEQ ID NO: 15213 - RNA, 2541 nt, Homo sapiens
  source 1..2541: mol_type = other RNA
gctgggattacaggcatgagccactgcacttcgccccctgcctcttctaagaagcttccgccgcttaatccctccattggcttcccactgcctggagcatctggctaactcttgcccttgtctggagggtagctgaagcacagctcccattttctcagctttcacacacgcaaggccatgtgtcctctgctctggccctctgcctgtctgcccagggcagagcccagcacgaggctggcccagctggatatgcatggagcatacctgggttgcattaaagtgctccccacttctgcttgccaagttcccactcagccctcaacatctggctcagatgctccctcctcagagagctctttcctgactccttggactgggtcatgggcactgtctgtgtaccccctccccccagccatgcttccctctgtcacaaccctgatgttgctgtgccagtctgtacttccagcagttgggagcccgtatggaccagggctaggactggttcttctagggccccagaaccaacacaggcctgagcacaaggtgtcagtaaaggctttctaaataaatggaatatcactcctctccagagagctcataatcatccctcaaaacccagctcaaatgccccttcccagaagctctcacctccccctctcatcttccctcacccgcttcattggtgactcaaagcatggagcataccccttgatgacagtacacgtcacactgtatttttgtgagcaccttaatgtggtttccccagctctccatggctgactgggacctctcaagagccaggcccaggtctgtccatctccatgcccacagggtctgggccagagaaggggctgaagaaatagtttttggtgagcttctgggtcctgtgagggatcttaactccatgcccagctgagctgaactctaattctccgcatggtttggggttggtggggctcctggtgccccggacacaatggcaaatatgaaggctgcccaggacctggaggactcagcgaccctgcctctgccatttggctgtgagtttctgtaggagctcatgtggtcgccggcggaacttcttctgggtgaagtagaagaggatggggtccagcacgctgttggcactggcaaacggccgcgtgcctttgtaggccgctgcaaaggcctccaatacagtgcaggggacgcccggcgtcgagcgcactgccaggtaggctgtcttggtgatgtgaaaaggcaggaagctgatggcaaaggcagcagccaccaccacggccatgcgggccgccttgccacgccgctcctgggccacaggctctgccgggccatcctggcggcacaggcggcaggccaggagacagtagcaggccagcagggcagcaaagggcagcaggaagccgatgacagtgagagccatgccatagggcatatagtgggtggccagggcaggcgggctgaggtcatagcagacagtgcggttacgctggatgcctgtggcagcgaagatggctgtgggcaggcactgggttgtcacggccagccacacggctacacacactagccaggcagcccggcggcccccacgtttgtgccagggggccagcgggtggcagatgcccaggtagcgctggaagctgatgcaggtgaggaagaggatgctgccgtgcaggttggcatagaagaggaagcggaccaggcggcaggcgaagtcgccaaagggccagtgatcaccttgggcatagttgtagatgagcaggggcagggagcaggcatatagcaggtcagccagagcaaggtttagggtgtacacggccgtgcgggtcagggcccggcgggacgtgcagatctgggtaatgacacagatgttcagcggcaggccagccgccagcaccgccgaatacacaggtggcagcagcagttgcttgaagttctcgcggtagacacaggtggtgggtggcaagcccagagcctggcctgtgccattgtcccattccatggctgcccaggtgggtttcctatgttcagggaggcaggggctcactgaggaccgcacccatctcctcagcctgaactccgccttccaaagccatggttcttctggcagaggtcttgttatccaagagttagcaagtgcctcgcttgcagtccgtgaagtgctggagcaaattcccactcgtggagcagcccctgctgccagtcagttctgtgcctgaaactgtcgcgtgcaatgttctggcagaagtctggagaggcagcagatgaggaaaccgagagacatatcaggagtgtcatgaagaatgagcaagacactgacaagaaggcagtttgcaaatttttagacactatccagatgacaggcaagcagaaaactcatctgaaaaccagcccctcatcctgtggggccctgaggtagccccagagcaggtccttgatccttgatgggaaataagcacaaattccacagaaccagttcttccgaaaagacaaagccacctctgctcccagccagctgacaggaagggcccctcctctgtcctt

SEQ ID NO: 15214 - RNA, 2423 nt, Homo sapiens
  source 1..2423: mol_type = other RNA
gctgggattacaggcatgagccactgcacttcgccccctgcctcttctaagaagcttccgccgcttaatccctccattggcttcccactgcctggagcatctggctaactcttgcccttgtctggagggtagctgaagcacagctcccattttctcagctttcacacacgcaaggccatgtgtcctctgctctggccctctgcctgtctgcccagggcagagcccagcacgaggctggcccagctggatatgcatggagcatacctgggttgcattaaagtgctccccacttctgcttgccaagttcccactcagccctcaacatctggctcagatgctccctcctcagagagctctttcctgactccttggactgggtcatgggcactgtctgtgtaccccctccccccagccatgcttccctctgtcacaaccctgatgttgctgtgccagtctgtacttccagcagttgggagcccgtatggaccagggctaggactggttcttctagggccccagaaccaacacaggcctgagcacaaggtgtcagtaaaggctttctaaataaatggaatatcactcctctccagagagctcataatcatccctcaaaacccagctcaaatgccccttcccagaagctctcacctccccctctcatcttccctcacccgcttcattggtgactcaaagcatggagcataccccttgatgacagtacacgtcacactgtatttttgtgagcaccttaatgtggtttccccagctctccatggctgactgggacctctcaagagccaggcccaggtctgtccatctccatgcccacagggtctgggccagagaaggggctgaagaaatagtttttggtgagcttctgggtcctgtgagggatcttaactccatgcccagctgagctgaactctaattctccgcatggtttggggttggtggggctcctggtgccccggacacaatggcaaatatgaaggctgcccaggacctggaggactcagcgaccctgcctctgccatttggctgtgagtttctgtaggagctcatgtggtcgccggcggaacttcttctgggtgaagtagaagaggatggggtccagcacgctgttggcactggcaaacggccgcgtgcctttgtaggccgctgcaaaggcctccaatacagtgcaggggacgcccggcgtcgagcgcactgccaggtaggctgtcttggtgatgtgaaaaggcaggaagctgatggcaaaggcagcagccaccaccacggccatgcgggccgccttgccacgccgctcctgggccacaggctctgccgggccatcctggcggcacaggcggcaggccaggagacagtagcaggccagcagggcagcaaagggcagcaggaagccgatgacagtgagagccatgccatagggcatatagtgggtggccagggcaggcgggctgaggtcatagcagacagtgcggttacgctggatgcctgtggcagcgaagatggctgtgggcaggcactgggttgtcacggccagccacacggctacacacactagccaggcagcccggcggcccccacgtttgtgccagggggccagcgggtggcagatgcccaggtagcgctggaagctgatgcaggtgaggaagaggatgctgccgtgcaggttggcatagaagaggaagcggaccaggcggcaggcgaagtcgccaaagggccagtgatcaccttgggcatagttgtagatgagcaggggcagggagcaggcatatagcaggtcagccagagcaaggtttagggtgtacacggccgtgcgggtcagggcccggcgggacgtgcagatctgggtaatgacacagatgttcagcggcaggccagccgccagcaccgccgaatacacaggtggcagcagcagttgcttgaagttctcgcggtagacacaggtggtgggtggcaagcccagagcctggcctgtgccattgtcccattccatggctgcccaggtgggtttcctatgttcagggaggcaggggctcactgaggaccgcacccatctcctcagcctgaactccgccttccaaagccatggttcttctggcagaggtcttgttatccaagagttagcaagtgcctcgcttgcagtccgtgaagtgctggagcaaattcccactcgtggagcagcccctgctgccagtcagttctgtgcctgaaactgtcgcgtgcaatgttctggcagaagtctggagaggcagcagatgaggaaaccgagagacctgcgccgcgcagcaccagctggtccggcccagatgtcactcgcccaggcgctgctaggaggcgaacccgtcaaatgaggggaccgtgtagacggcggcagcagctccggccccagcgtccctggaacccagaggagccagagc

SEQ ID NO: 15215 - RNA, 2355 nt, Homo sapiens
  source 1..2355: mol_type = other RNA
gctgggattacaggcatgagccactgcacttcgccccctgcctcttctaagaagcttccgccgcttaatccctccattggcttcccactgcctggagcatctggctaactcttgcccttgtctggagggtagctgaagcacagctcccattttctcagctttcacacacgcaaggccatgtgtcctctgctctggccctctgcctgtctgcccagggcagagcccagcacgaggctggcccagctggatatgcatggagcatacctgggttgcattaaagtgctccccacttctgcttgccaagttcccactcagccctcaacatctggctcagatgctccctcctcagagagctctttcctgactccttggactgggtcatgggcactgtctgtgtaccccctccccccagccatgcttccctctgtcacaaccctgatgttgctgtgccagtctgtacttccagcagttgggagcccgtatggaccagggctaggactggttcttctagggccccagaaccaacacaggcctgagcacaaggtgtcagtaaaggctttctaaataaatggaatatcactcctctccagagagctcataatcatccctcaaaacccagctcaaatgccccttcccagaagctctcacctccccctctcatcttccctcacccgcttcattggtgactcaaagcatggagcataccccttgatgacagtacacgtcacactgtatttttgtgagcaccttaatgtggtttccccagctctccatggctgactgggacctctcaagagccaggcccaggtctgtccatctccatgcccacagggtctgggccagagaaggggctgaagaaatagtttttggtgagcttctgggtcctgtgagggatcttaactccatgcccagctgagctgaactctaattctccgcatggtttggggttggtggggctcctggtgccccggacacaatggcaaatatgaaggctgcccaggacctggaggactcagcgaccctgcctctgccatttggctgtgagtttctgtaggagctcatgtggtcgccggcggaacttcttctgggtgaagtagaagaggatggggtccagcacgctgttggcactggcaaacggccgcgtgcctttgtaggccgctgcaaaggcctccaatacagtgcaggggacgcccggcgtcgagcgcactgccaggtaggctgtcttggtgatgtgaaaaggcaggaagctgatggcaaaggcagcagccaccaccacggccatgcgggccgccttgccacgccgctcctgggccacaggctctgccgggccatcctggcggcacaggcggcaggccaggagacagtagcaggccagcagggcagcaaagggcagcaggaagccgatgacagtgagagccatgccatagggcatatagtgggtggccagggcaggcgggctgaggtcatagcagacagtgcggttacgctggatgcctgtggcagcgaagatggctgtgggcaggcactgggttgtcacggccagccacacggctacacacactagccaggcagcccggcggcccccacgtttgtgccagggggccagcgggtggcagatgcccaggtagcgctggaagctgatgcaggtgaggaagaggatgctgccgtgcaggttggcatagaagaggaagcggaccaggcggcaggcgaagtcgccaaagggccagtgatcaccttgggcatagttgtagatgagcaggggcagggagcaggcatatagcaggtcagccagagcaaggtttagggtgtacacggccgtgcgggtcagggcccggcgggacgtgcagatctgggtaatgacacagatgttcagcggcaggccagccgccagcaccgccgaatacacaggtggcagcagcagttgcttgaagttctcgcggtagacacaggtggtgggtggcaagcccagagcctggcctgtgccattgtcccattccatggctgcccaggtgggtttcctatgttcagggaggcaggggctcactgaggaccgcacccatctcctcagcctgaactccgccttccaaagccatggttcttctggcagaggtcttgttatctccaagacttgagccaactcattggatggtaatttatcagaacagtgtttttatatgcagaaatattatagaagaatgcaaaatccacaggaattttggaagataaaaaaatgagatttcggagcagcttctcttgtatgtgcatgtgtttgtatgtgtgagagggtgagcctgggacctgtcatactttctccacccagatccgggtgagctttcactctcccaagccctcccg

SEQ ID NO: 15216 - RNA, 2263 nt, Homo sapiens
  source 1..2263: mol_type = other RNA
gctgggattacaggcatgagccactgcacttcgccccctgcctcttctaagaagcttccgccgcttaatccctccattggcttcccactgcctggagcatctggctaactcttgcccttgtctggagggtagctgaagcacagctcccattttctcagctttcacacacgcaaggccatgtgtcctctgctctggccctctgcctgtctgcccagggcagagcccagcacgaggctggcccagctggatatgcatggagcatacctgggttgcattaaagtgctccccacttctgcttgccaagttcccactcagccctcaacatctggctcagatgctccctcctcagagagctctttcctgactccttggactgggtcatgggcactgtctgtgtaccccctccccccagccatgcttccctctgtcacaaccctgatgttgctgtgccagtctgtacttccagcagttgggagcccgtatggaccagggctaggactggttcttctagggccccagaaccaacacaggcctgagcacaaggtgtcagtaaaggctttctaaataaatggaatatcactcctctccagagagctcataatcatccctcaaaacccagctcaaatgccccttcccagaagctctcacctccccctctcatcttccctcacccgcttcattggtgactcaaagcatggagcataccccttgatgacagtacacgtcacactgtatttttgtgagcaccttaatgtggtttccccagctctccatggctgactgggacctctcaagagccaggcccaggtctgtccatctccatgcccacagggtctgggccagagaaggggctgaagaaatagtttttggtgagcttctgggtcctgtgagggatcttaactccatgcccagctgagctgaactctaattctccgcatggtttggggttggtggggctcctggtgccccggacacaatggcaaatatgaaggctgcccaggacctggaggactcagcgaccctgcctctgccatttggctgtgagtttctgtaggagctcatgtggtcgccggcggaacttcttctgggtgaagtagaagaggatggggtccagcacgctgttggcactggcaaacggccgcgtgcctttgtaggccgctgcaaaggcctccaatacagtgcaggggacgcccggcgtcgagcgcactgccaggtaggctgtcttggtgatgtgaaaaggcaggaagctgatggcaaaggcagcagccaccaccacggccatgcgggccgccttgccacgccgctcctgggccacaggctctgccgggccatcctggcggcacaggcggcaggccaggagacagtagcaggccagcagggcagcaaagggcagcaggaagccgatgacagtgagagccatgccatagggcatatagtgggtggccagggcaggcgggctgaggtcatagcagacagtgcggttacgctggatgcctgtggcagcgaagatggctgtgggcaggcactgggttgtcacggccagccacacggctacacacactagccaggcagcccggcggcccccacgtttgtgccagggggccagcgggtggcagatgcccaggtagcgctggaagctgatgcaggtgaggaagaggatgctgccgtgcaggttggcatagaagaggaagcggaccaggcggcaggcgaagtcgccaaagggccagtgatcaccttgggcatagttgtagatgagcaggggcagggagcaggcatatagcaggtcagccagagcaaggtttagggtgtacacggccgtgcgggtcagggcccggcgggacgtgcagatctgggtaatgacacagatgttcagcggcaggccagccgccagcaccgccgaatacacaggtggcagcagcagttgcttgaagttctcgcggtagacacaggtggtgggtggcaagcccagagcctggcctgtgccattgtcccattccatggctgcccaggtgggtttcctatgttcagggaggcaggggctcactgaggaccgcacccatctcctcagcctgaactccgccttccaaagccatggttcttctggcagaggtcttgttatctgcgccgcgcagcaccagctggtccggcccagatgtcactcgcccaggcgctgctaggaggcgaacccgtcaaatgaggggaccgtgtagacggcggcagcagctccggccccagcgtccctggaacccagaggagccagagc

SEQ ID NO: 15217 - RNA, 2337 nt, Homo sapiens
  source 1..2337: mol_type = other RNA
gctgggattacaggcatgagccactgcacttcgccccctgcctcttctaagaagcttccgccgcttaatccctccattggcttcccactgcctggagcatctggctaactcttgcccttgtctggagggtagctgaagcacagctcccattttctcagctttcacacacgcaaggccatgtgtcctctgctctggccctctgcctgtctgcccagggcagagcccagcacgaggctggcccagctggatatgcatggagcatacctgggttgcattaaagtgctccccacttctgcttgccaagttcccactcagccctcaacatctggctcagatgctccctcctcagagagctctttcctgactccttggactgggtcatgggcactgtctgtgtaccccctccccccagccatgcttccctctgtcacaaccctgatgttgctgtgccagtctgtacttccagcagttgggagcccgtatggaccagggctaggactggttcttctagggccccagaaccaacacaggcctgagcacaaggtgtcagtaaaggctttctaaataaatggaatatcactcctctccagagagctcataatcatccctcaaaacccagctcaaatgccccttcccagaagctctcacctccccctctcatcttccctcacccgcttcattggtgactcaaagcatggagcataccccttgatgacagtacacgtcacactgtatttttgtgagcaccttaatgtggtttccccagctctccatggctgactgggacctctcaagagccaggcccaggtctgtccatctccatgcccacagggtctgggccagagaaggggctgaagaaatagtttttggtgagcttctgggtcctgtgagggatcttaactccatgcccagctgagctgaactctaattctccgcatggtttggggttggtggggctcctggtgccccggacacaatggcaaatatgaaggctgcccaggacctggaggactcagcgaccctgcctctgccatttggctgtgagtttctgtaggagctcatgtggtcgccggcggaacttcttctgggtgaagtagaagaggatggggtccagcacgctgttggcactggcaaacggccgcgtgcctttgtaggccgctgcaaaggcctccaatacagtgcaggggacgcccggcgtcgagcgcactgccaggtaggctgtcttggtgatgtgaaaaggcaggaagctgatggcaaaggcagcagccaccaccacggccatgcgggccgccttgccacgccgctcctgggccacaggctctgccgggccatcctggcggcacaggcggcaggccaggagacagtagcaggccagcagggcagcaaagggcagcaggaagccgatgacagtgagagccatgccatagggcatatagtgggtggccagggcaggcgggctgaggtcatagcagacagtgcggttacgctggatgcctgtggcagcgaagatggctgtgggcaggcactgggttgtcacggccagccacacggctacacacactagccaggcagcccggcggcccccacgtttgtgccagggggccagcgggtggcagatgcccaggtagcgctggaagctgatgcaggtgaggaagaggatgctgccgtgcaggttggcatagaagaggaagcggaccaggcggcaggcgaagtcgccaaagggccagtgatcaccttgggcatagttgtagatgagcaggggcagggagcaggcatatagcaggtcagccagagcaaggtttagggtgtacacggccgtgcgggtcagggcccggcgggacgtgcagatctgggtaatgacacagatgttcagcggcaggccagccgccagcaccgccgaatacacaggtggcagcagcagttgcttgaagttctcgcggtagacacaggtggtgggtggcaagcccagagcctggcctgtgccattgtcccattccatggctgcccaggtgggtttcctatgttcagggaggccaagagttagcaagtgcctcgcttgcagtccgtgaagtgctggagcaaattcccactcgtggagcagcccctgctgccagtcagttctgtgcctgaaactgtcgcgtgcaatgttctggcagaagtctggagaggcagcagatgaggaaaccgagagacctgcgccgcgcagcaccagctggtccggcccagatgtcactcgcccaggcgctgctaggaggcgaacccgtcaaatgaggggaccgtgtagacggcggcagcagctccggccccagcgtccctggaacccagaggagccagagc

SEQ ID NO: 15218 - RNA, 2358 nt, Homo sapiens
  source 1..2358: mol_type = other RNA
gctgggattacaggcatgagccactgcacttcgccccctgcctcttctaagaagcttccgccgcttaatccctccattggcttcccactgcctggagcatctggctaactcttgcccttgtctggagggtagctgaagcacagctcccattttctcagctttcacacacgcaaggccatgtgtcctctgctctggccctctgcctgtctgcccagggcagagcccagcacgaggctggcccagctggatatgcatggagcatacctgggttgcattaaagtgctccccacttctgcttgccaagttcccactcagccctcaacatctggctcagatgctccctcctcagagagctctttcctgactccttggactgggtcatgggcactgtctgtgtaccccctccccccagccatgcttccctctgtcacaaccctgatgttgctgtgccagtctgtacttccagcagttgggagcccgtatggaccagggctaggactggttcttctagggccccagaaccaacacaggcctgagcacaaggtgtcagtaaaggctttctaaataaatggaatatcactcctctccagagagctcataatcatccctcaaaacccagctcaaatgccccttcccagaagctctcacctccccctctcatcttccctcacccgcttcattggtgactcaaagcatggagcataccccttgatgacagtacacgtcacactgtatttttgtgagcaccttaatgtggtttccccagctctccatggctgactgggacctctcaagagccaggcccaggtctgtccatctccatgcccacagggtctgggccagagaaggggctgaagaaatagtttttggtgagcttctgggtcctgtgagggatcttaactccatgcccagctgagctgaactctaattctccgcatggtttggggttggtggggctcctggtgccccggacacaatggcaaatatgaaggctgcccaggacctggaggactcagcgaccctgcctctgccatttggctgtgagtttctgtaggagctcatgtggtcgccggcggaacttcttctgggtgaagtagaagaggatggggtccagcacgctgttggcactggcaaacggccgcgtgcctttgtaggccgctgcaaaggcctccaatacagtgcaggggacgcccggcgtcgagcgcactgccaggtaggctgtcttggtgatgtgaaaaggcaggaagctgatggcaaaggcagcagccaccaccacggccatgcgggccgccttgccacgccgctcctgggccacaggctctgccgggccatcctggcggcacaggcggcaggccaggagacagtagcaggccagcagggcagcaaagggcagcaggaagccgatgacagtgagagccatgccatagggcatatagtgggtggccagggcaggcgggctgaggtcatagcagacagtgcggttacgctggatgcctgtggcagcgaagatggctgtgggcaggcactgggttgtcacggccagccacacggctacacacactagccaggcagcccggcggcccccacgtttgtgccagggggccagcgggtggcagatgcccaggtagcgctggaagctgatgcaggtgaggaagaggatgctgccgtgcaggttggcatagaagaggaagcggaccaggcggcaggcgaagtcgccaaagggccagtgatcaccttgggcatagttgtagatgagcaggggcagggagcaggcatatagcaggtcagccagagcaaggtttagggtgtacacggccgtgcgggtcagggcccggcgggacgtgcagatctgggtaatgacacagatgttcagcggcaggccagccgccagcaccgccgaatacacaggtggcagcagcagttgcttgaagttctcgcggtagacacaggtggtgggtggcaagcccagagcctggcctgtgccattgtcccattccatggctgcccaggtgggtttcctatgttcagggaggccaagagttagcaagtgcctcgcttgcagtccgtgaagtgctggagcaaattcccactcgtggagcagcccctgctgccagtcagttctgtgcctgaaactgtcgcgtgcaatgttctggcagaagtctggagaggcagcagatgaggaaaccgagagacctggggagaggaagtaacttgccacagcacagagctggcaagcagcagggccaggactcgaatcccgagaaccctgaagctccagtcctttacaccaatgctgactcatcctctacccagctgcccgcaagtcacttcattcaccctctgtttgctcactcaaac

SEQ ID NO: 15219 - RNA, 88 nt, Homo sapiens
  source 1..88: mol_type = other RNA
gctgggattacaggcatgagccactgcacttggtcggagtttcacattttcaaggaactatacttgtagtttttgagtggaaacaagg

SEQ ID NO: 15220 - RNA, 383 nt, Homo sapiens
  source 1..383: mol_type = other RNA
gctgggattacaggcatgagccactgcagctagccttgcctttctgattcaagggttcaattgttaagctgtcggggccaatatccacaatattgcccatctgaaatccatctgtagggtgtggcgcccaaacgggctttccatcctccatttttgaaggaggatccacgatctcctgtttccactatccactgtcaccggtgcgggagcgaaggcaggtgcgcggcggcggggctacctgtacgggtgaagctggagggcgcggtgagaagtgatgagggccagtgaagagggcgacgacgcggacgggcaccaggacagggcggcgacagcggccgggctgaggctggcttcctgctcggacagatcccgagtcggtctcc

SEQ ID NO: 15221 - RNA, 3373 nt, Homo sapiens
  source 1..3373: mol_type = other RNA
gctgggattacaggcatgagccactgcagtcagccagtaaggatcactcttatccctagtaaaaaggatccgtgatacaaaatggccactgagtcccttctctctccccagtctcttacacattctcataaacagtgattgactcacttattttctgcagaagacagaatggcatgaatgggacggaaacggttcatatgactacttggatatctctcatcctgtgaaccagtctaacaagcaattaccttgaggaatctggaaaagcatgtggattgggcgatcctctcttaaggcacttagaacagagaatgtgcacggtgtagtgcagtccaggccattcctgaagtaggacattcagttcctccaccaagggggttatggcttgccatgcggtccatatatttggtaatgatgcatggctagcaatggacagggtgtctggctgcaggactcccctggcaggtctgtaactcacaaccacaggaactttccctctataggcaaagatctgaaatttaccatccgacctgtgcaccacatggctgttgatctggacactgtagcgtgcaaacaacccaagtggaaaagtaaaaggaaagctatattcaatctgcaactgctcagccacaaaagactgcccagctaggttggtcccattaatccaggcttctgcatggggcacctcgttctgcacatagcatgggaacttgtaccaagctgtggacccattcaaaggcttgcccttgggtttattgaggcagtaacagagtcccatcttctccagcagctccagcaacagctgcaagtcctgctgggcctggacatgaggcttaagcagcaaccgaatgacatgagctggcaagagcccatgcaacagaaagccctccacatactgatggagctgggtggcccggagcagttcctggctgggggtggaccgcgccatgggcggggagctttccccctccgccttgccctctccactggtccctaggagcagcttatgcagcagcaaagagggatccctctggaagaagacattgaggatgtcgatgaggcgggtgaggttgtggaagacgtgctccttgagagccggactgtcctcaaagtagagtagcttgccgctctcatgcaggtaggagagggcactctgcagtcggtcctcggtcagacccgcctgcaggcccaagcgcgccgagtcccaccagcttagccacagtcgctgggcctgaggtggctggaaatgcagttcctccagcacctgccaggatcgaggcagtactctgtgtaagttggggaagatctctcggtgctcagcaactgacagcaacttgtcccgaaggcgtcgtaagtggcgcgggtccctgcagctaacaggcaacacgggggagaggatctgcagccggtggttgagcaggtattgaaaatgggccttgcgccgtcgaaggttcttgtccgaaacgccatagtaggctgcgtgggggctggcagagcgcagctcgaagtcccgggccagtgcctcgtccaccaccttggccaagcggctcagtccctccgcgtcgtgcttctcctgcagggcgatctggcggtgaatgtccagacatttctcctccagctcacgctctccgcacaggtctgcgtgggtgcccacgatgcacaccaccgcgtggggcactctcgccccgacccgatgcaagaaggagcccacggtggtaggaaagtggcgaggctcataggtggccaagttgaccaccagcacgtatagggcccctggggacaggaagaagggctggatcacctcataactttcatccccagctaagtcatacacgatgaaccgcaggccccgggaggcatcggccgtccagctggtcacctcgatgcccttgctcacagggggaggtgacggtgggtagcacttctccttgtcccctcctcctgggcatccctccactctctcctcggtgaggcagtggcgcagcaaagtctttcctgcagccttatgccccatcaggagcagcttgagccggggctgcaccgccggctgggaatgagccagttccttctggtaggctgcgatgtaggggatccccttcatgcagacctcgtaggggggctggatcagtgggttgtctttgatcttccacaaacccacccgggagagctggccaaagtggtcgggcagcaccgcgatctggttcccctgcagcacgagctcctccaggccggtcagctccacgatggagtccggcaggtagcggatgcggttattatccagccacaaggtgagaagccggcccaggcccgagataagggatggcaccgaggtgagctggttgcgactaaggtagagctcctccagaccagccaggggcagcagcgcggcagggaactcctcgaagaggttggaggagaggttgagcattttgagccgctgcaggcagctgaactgggcgggcagagcctgcagcccgttgttgtctagcatgaggctctccaaactggccagctcgcagaagccggcgggcagcgtgccaagctcggccccactcagccagaggatcttgagggcacgcagggcactgatatcctcaggcaggccccgcagccggttgctggacacgtccagctcctccagggccaccagctgcagcagctgccgggggaaggcagtgagctggttgtgatccacgtccagggtgcgcaggcgggagaggcaggagagggagtcaggcaggtgcgccagccggttaaagctgacatccagctcctccaggtgagcgagagcgcccagctgggcgggcagggcgggcagctggttgtggctgaggttgagcttccgcagctccctcagagcactcaccacctccgcgcccagggcggtcagccggttgtggctcacgtccagctcggtgaggtggtggccgagctcggccaccgccgggggcagccgggcgaagcggttcctgcgcaggaccaggacgcgcaggctgcccagcgccgaccccagcccctcgggtacctcctccaggccgttgttccccaggttcagtgcctcaatgtccccgaggttggccggcagcacgagctggggggaggcgggggactcgagcgcgtcggccccggccccggggcaggccccggcggcggtaagcgtgagctggcgcaggttgctccgcagcttcctggcacgcagggcggcgtcccgccacagcctcgcggtcttcaggttgccactgtccatcccagccatggcggggccccgggccgacagcctcacgcggacgcgggagcccgcagctacatgccgcgccgcgccccgggccctccggctcctgcccctgcctgccctcccgcgctcggcggccgg

SEQ ID NO: 15222 - RNA, 2733 nt, Homo sapiens
  source 1..2733: mol_type = other RNA
gctgggattacaggcatgagccactgcatcagaagtctctgtccatgtgtgagggtgacactcaacttttggcaggatgagcatacaagagtcacaatctcacctgtgtgctgggtgcagttatatgtcaaaatcccacctgagtcacagtatcaatgatgaactggatccatgcatgagagtcccaattccacctgtagactgtgtgttgtgttggccctatgatatgtcacaatccacctccatttgcataacctagagaaaatagaagagtcgcagagccttctgtgactcgtattagagtcaaagccttctagttgtgttgaatcctggtcttagagtcaccatccacctggaatatgtctcaatctcccctgtgggcaaggcccaggctggagaatcagatcacttgcatgcagggcccagtgacatattatattttctctaggcacagcccaggcaggagagtcacaacatttgggtgttgggctcagagatatgtcataatccctttttgggtcatgtctcctaggtgagaagatcagagatgttgccgattctgtgtaagtctcaggaataagagaagagtcaggtatcctagaaactcggctacattatatgttgcaattacccaagtgggcaggaatctcatgagaagagggtcacatcatgtagctgctgagctaaacgatgcatcacaattcccactgtgtattggtcccagaaagaagaggagagtctcatcatctaggtgatgggcctggaaatctggcatatgcatcctaggtgctggatccagtgatatgtcacaatcctcttctttggcatggcacaggaagaagtagagagtcacaccacctaggtgttggaccaagccatatgtcacaatacacaataaatgcagggcctaggtgcttggtccagtaatatgtcaaaattcccttgagaggtgagcccaggcaagagagtcacatcatttcggtgagaaccccacagatgtgtcactattttccctgtgaatagcgctgtgtgctgggcccagtgataagtcactttcccttgtgtgggcatggcttcagcaggagagaagagtcacatcaccaaggttctggttccagagatatgtcacaatctctccttgatgttggacccagccatatatcacaatgcacagcatatccagggctcaagcagggaagaaaaatcacatcgtctagttgctgggtttgatgatatgtcacaatcacttgtttttgcagaacccagacagaaaagaagagtcacatctcctagttcatggatgcagagataagccaaaaggctccttgtgggcaggacccaggcacaaggctctcatgccctaggtgtttgtctcagccatacgtcacattaccaaatatatgcagggcccaggcaaacaaggtgagtcataacaccttggtactaagtttaatgatatgttacaatccccacttttggcagggccaggacgcacacacacacacacacacaaacaaaggcacatcacataggtgattaaaaaaaaaagatatgtcataatatccctgtaagcagggctcatgcataagagtctcatcacctaggttttagacccagagatttgtcacaatacacaatttatgcaagactcagacacaagaggaaagtcacgtaacctaggtgctgggtccagtgatacattagaatctctccttgggtagagtccaagcagtagaaaagagttacattacctgggtacttgctccaggaatatgtcacaatacctcctgtgtgtgaggtccagtgataagccactcttccttttgtgcacacggtccaaacaaaagatgaaagtcacatcacctaggtgctgggcttccagaattgtctcaatccctcagacaattgttgtcttgattcgatcctcttcaagaggtgatttatggtccgctatggaactttgccaggtatttttaaatgcaggtttctgataactttggagactgtcggtaggaagtgagcagcagattcacatcatgtaggttttcggcaaagatatgtcacaatctttcctgaggtcagaaaccacgcagaagtcatctcacctaggtgctcagccacagatatattacaatcccctcttaaagcagagtacaggcagcagagtcatttcacctgggtgctgagcccagtgatatgtcaaaatgctctctgtgggcacagccttggcaggagagacacatcatctggtgactgggtccagcaatacattacaacattttctgcgacatgggacatgtaacctgtgagtaggtagtgagcaggagagtcacatcaactgggtgcttggccagagatttgtacaatattccctgatggaagggaccaggcaggagaggaacatcacctgggtgctgagcccagtggcatgtcacaatgctccctcaactaggttctgggtccagtgaattgctacaatctccttttttctttggcagtgcccaggcagaagagaagaggcaaataacaatctcaactgtggacttgatctgtgtatgagaccttccatccatcctctagactgtgtctccttagtggactcacggtttctcaagtctcaggggtgctgaatcttggtctgagagttaccagcttacttgtacactggattcaaggatgaaagtcaatttttcaacttttgaaactttcattggttttgagattcagaatctc

SEQ ID NO: 15223 - RNA, 1911 nt, Homo sapiens
  source 1..1911: mol_type = other RNA
gctgggattacaggcatgagccactgcatccagcatgcacgtctctttcattgactgtttctgagatgtatccttcacaatgaaccagtaataggaaatgaactggccagatgtggtggctcacatctgtaatcccagcactttcagaggctgaggtgggaggatcacttgagaccaggaatttgtggccagcctggccaacacaacaagaccccatctatacaaaaaataaaagaaactagccagatgtggtggtgcaggcatgtagtctcagctactagggaggctgaggtgggagaaccactggaacccagacaatcaaggctgcaatgagctatgactgcaccattgcacaccagcctgggcaacaaaataagaccctctctctcagaaaaaaagaaaataaactgtttttctgagttccgtaaactgttctagcaaattattaaacccaagaagacagttacgggaacccccgattggtaacaggttggtcaaaagtatggtgacaacttaggacttgccattgtcatctgaagtgaggatggcctcgtgggactgagcccctaacttgtggggtctgtgctaactccaggtagtgtcagaataaagtcatgggatacccagttaatatccagagcactgaagaatctggtgtagaaactccatacatacattcagtcggaagtgtgtgagtagagacaaacatgggcttttctgtcacctacctgcttaactgcataggagaggcaatatgtggtgctcatgaacaaagcaaacattaaagtcagaccagacccaacatttgactcagtcttaatatccaggtgagcctgcgcaaatcattcattattcctaaggttttcatcactccattcataaaatggggataactgtggcacctacatgtgattctgtgagaattaacaaaatattatgcttggggttattgtgatcattatacctgttccaaactatttgacaaggacagtgatggatgaagacatcaaaaaatcagaaactgcaatgaggtctctcaggcaaaattccatacaagcaaattactgtgtctacaaagcattcctgccacacttaattcaccattccctgaacaaaatatgccatcttcattgttcaggtctgtacagtgctggtgtcccttcccgggcagtttgcgctatcccatcccggcccattccccatccctccacctcccccttccctccccactctcatacaactcttcctcatctttcaggacttggcttcaatgtcaccttaactggaagcttctctcactctccagaagagcttcccattgcacctgatgcatgggaaacataatttgatcatttttaagttacagtccaaatctttttgtacctgaataacatgttgcccagtcagtctctcttcctggattcacaagtctttcatggtagatccagctccagctctgtggccctgtggttggagaccgctgctcaagtgcatttgaaaggaaccatcccacgccattcttcagagtcatctttactgctgcagtggtcaacttgtagcacccctaagcttgcaggacatatgcttcaactggcatttcacaatcaacagtatgtggcagcttgagtcattgtgagcgcacttcctggaaatcaccagcatcccatatcccattgcaaggagctcagcactgctccttggataaccaaacctattcccaaatcccatctgtgtgcgtctatctcctggtacccttcctagcatcaattctgtatttgtaggagtccaatcaggagacacaaaccactcaaaagtttaaactagaatgagcaagatggctcacacctgtaatcccagaactctgggaggccaaggtgggtggactgctttgagctcaggagtttgagaaca

SEQ ID NO: 15224 - RNA, 1968 nt, Homo sapiens
  source 1..1968: mol_type = other RNA
gctgggattacaggcatgagccactgcatccagcatgcacgtctctttcattgactgtttctgagatgtatccttcacaatgaaccagtaataggaaatgaactggccagatgtggtggctcacatctgtaatcccagcactttcagaggctgaggtgggaggatcacttgagaccaggaatttgtggccagcctggccaacacaacaagaccccatctatacaaaaaataaaagaaactagccagatgtggtggtgcaggcatgtagtctcagctactagggaggctgaggtgggagaaccactggaacccagacaatcaaggctgcaatgagctatgactgcaccattgcacaccagcctgggcaacaaaataagaccctctctctcagaaaaaaagaaaataaactgtttttctgagttccgtaaactgttctagcaaattattaaacccaagaagacagttacgggaacccccgattggtaacaggttggtcaaaagtatggtgacaacttaggacttgccattgtcatctgaagtgaggatggcctcgtgggactgagcccctaacttgtggggtctgtgctaactccaggtagtgtcagaataaagtcatgggatacccagttaatatccagagcactgaagaatctggtgtagaaactccatacatacattcagtcggaagtgtgtgagtagagacaaacatgggcttttctgtcacctacctgcttaactgcataggagaggcaatatgtggtgctcatgaacaaagcaaacattaaagtcagaccagacccaacatttgactcagtcttaatatccaggtgagcctgcgcaaatcattcattattcctaaggttttcatcactccattcataaaatggggataactgtggcacctacatgtgattctgtgagaattaacaaaatattatgcttggggttattgtgatcattatacctgttccaaactatttgacaaggacagtgatggatgaagacatcaaaaaatcagaaactgcaatgaggtctctcaggcaaaattccatacaagcaaattactgtgtctacaaagcattcctgccacacttaattcaccattccctgaacaaaatatgccatcttcattgttcaggtctgtacagtgctggtgtcccttcccgggcagtttgcgctatcccatcccggcccattccccatccctccacctcccccttccctccccactctcatacaactcttcctcatctttcaggacttggcttcaatgtcaccttaactggaagcttctctcactctccagaagagcttcccattgcacctgatgcatgggaaacataatttgatcatttttaagttacagtccaaatctttttgtacctgaataacatgttgcccagtcagtctctcttcctggattcacaagtctttcatggtagatccagtataatgtagactcagtgggatctctgagcttgttttcctgcaactagactgtccacctccagctctgtggccctgtggttggagaccgctgctcaagtgcatttgaaaggaaccatcccacgccattcttcagagtcatctttactgctgcagtggtcaacttgtagcacccctaagcttgcaggacatatgcttcaactggcatttcacaatcaacagtatgtggcagcttgagtcattgtgagcgcacttcctggaaatcaccagcatcccatatcccattgcaaggagctcagcactgctccttggataaccaaacctattcccaaatcccatctgtgtgcgtctatctcctggtacccttcctagcatcaattctgtatttgtaggagtccaatcaggagacacaaaccactcaaaagtttaaactagaatgagcaagatggctcacacctgtaatcccagaactctgggaggccaaggtgggtggactgctttgagctcaggagtttgagaaca

SEQ ID NO: 15225 - RNA, 3558 nt, Homo sapiens
  source 1..3558: mol_type = other RNA
gctgggattacaggcatgagccactgcatccagccaagttacccactcttaaggtattttgttataaccacctgaacaagaacaaagacattctctaagccatgtagtacacattcataaatctggggttttaaataccttcctcctataattgtcacgagggacagattcaagtttcatttggttgaagcttctaaacctggaaggaacctaaaatgagcttcagcttcaaggctaatgtgcctgttctccctccacgtaaagcagaaaatgccagatctcccttgccctgcttgctttgcagggaggatgtgactccacaatccaggttcccccaatctgtggccacacccaggatgaggatcagaagctagtgaccaccagcatcgctcctggtagctgatggcaacgtgagggaaactgcctcatttcacaggtaacagggtcagaagttctgttggcagccaacacagttcccagaccagctctgtgttccaatgtgacttgggttcatttatgtggctaactcaacttccctgtcctttccagaggttccatgagctcttcttttaaacatgtactgggcacttataggctctcatttcctgagctcgggactaaaccctctacacatccagcattcctttactaagcccctttgcccccagagctaggaggtgtggctcacaggcagggatcatcctctgctttcctccaaggcctggaccagaaggaccaagggaagacagttccagcccagagccatttcccttccaacctcttggcaagcctgatgagttccactccccgctgacgggcacacctgccttccaggcactgatcctgctttccccctcttgctctgccactcactgtgcctggcttgctgcccagccctccccagccttctctcctcctacctttcccacttattgcctccttccaggcttgtccagcatgataaactctggtctcagcattcacagcctcctctatctctcagctgtgtccctggtcatgactctgcttgctcttccctaaagcaattaaaataggaaaatctgacccttctcacccaggaggcaggtcctctcctatccactggagacccagagcaaaagctctctcctcccttcatcctccttctcaccatgtgatttcagacaagtcctttcacttccgagttttgccatgtgtgcctgtgtgcatatgtatgtgatgtacagacctctggagccatttcaccacagtgcctctccactcccagccagtgccagggcaccccctcagctgctgcaggatgtgtcaccagaaggagagagttaaaggggaagaaagcccttgagtaggagccaagtcatctgaacgcacaccctgtgcccagaggaggaggggcaagagttgctttccatgaagagtgcacctgatgagaaggcagctccagaggactcaaaggaaaaccaagaatcaagagagaaagaaacgtgcagtccttgcctacttggggagggggaggggtcgtaccacaaactccttggtcaatatagggacctgcttctccgtgcgccccagccccctctgcaccatgcactctcctcccgggcctagcgcctgctacaactgtggcctccactaatttcgggggtgcgaggcggtggatgatgcccaagtgaagccgttcaggcctcgtggcagcaccagatcaagggcgaggttgcgctgctcgtcctcagagtacacaggccggtagcccagcagctgcagcgcaccagcgcacagttcctgcacgcggcggatcttggcaaagggcagcgcatggcgccaggcctgggagacgttgagcgcattcctggacgaagtcttgaaggcttcgcggcgcgcaccaggtccagatccgtgggtgatgttatggatccaggcctcgagctgtggcgtgagactgagcccagtgaaggcgtagagcgcacggatttctgccagcggctcccgcgccaggtcctcgaagcgcaccaggcggtagcggccgcgcagaaagggtggcggcttgagtgtggcggcctcggcgatgcgtacgtggctacggcacacctcgcgcaccacgcgcaggccggggtcggcctccacccacgtgccgttggtgcccagcacgatgccgttgtcacgcgccagagccttggctgtctgctcccgggagcgcagcacggcccgcgggtcgcgcaccaggtgcacgatgcgtaggttgagcgcggggtcgctgagcagcgggtagagcacctgcaggttgaagaagcgcacctccttgagcaccacgtggctgtaggagcggcaggcctcccgggccagggtgaaggactgccgcgcgcacagtggcttgcacacggcctcgctgctgatggcgcctcggggaaaggcactgcaggcgggtggcgagcacagtgcacggctcacggcccactggaagaggtcggacaggttgcggcgccaaggcagataggcatcaaacacgtccatgtcgcacaggaagacggagcgcaccaggtcgcgcacagccatgtgcagcgttgcggcgctgccctgcgacagggtggtccacacgtgccacgcgggctccattaggtagaagacgtcggggtgctggttgaagagttggcccacgaaggacgagcccgagcgccacgaggacagcaccagcacatgcacgcgcgcctcgccgcctgctggggacgagggccctggccgggaaaccagaaagaggaggaggaaggtctgcgccaggaggagcgcggtcactgctgtgctggagacgcgcggcagccacatgctgactgctgggggccactgtccagggctgctgggagagctgcaacgctgatcacaaatccatgggagatgattagaggttcctcagcacaagtgttggtgagatgacagagacgtggggatcctcataaaatggggatgtcagatggtgcatttcctgaagaaacaatttggtggtttctcgaaaggttgaatagagtgaccatatgatacagcagatccactcctgggtacacaccctagagaacccaaagcttggcggctctgcccgagctgcagcggcacggtgggggacgcctctctccctggactcagcaaaggctcccaaacgtcgtctcttccaaattccaccgcacagccagctctttctcttcactgggagggtccgcaggggctgacttgctccttaaggtcccaagactattaagcgacacccggtgaggccgggaaaggggctctaagaggcatggacgagagttggcggtgaccaagccactggaagctcctggagactcgaggtagaacgaatgtgggaacagggcaggagtcccagaatgggatgttgaggctgggggtgtcctggggctaccacagggaaggacccggcgcagagctccctctggaacccggcactgcggcccgcgccctctactccccgcgcgccggccggcaaccctcggcgctgcccggtgcagcccgcccgagcgcacacaatgaggcgctttcagacgtggctgc

SEQ ID NO: 15226 - RNA, 3615 nt, Homo sapiens
  source 1..3615: mol_type = other RNA
gctgggattacaggcatgagccactgcatccagccaagttacccactcttaaggtattttgttataaccacctgaacaagaacaaagacattctctaagccatgtagtacacattcataaatctggggttttaaataccttcctcctataattgtcacgagggacagattcaagtttcatttggttgaagcttctaaacctggaaggaacctaaaatgagcttcagcttcaaggctaatgtgcctgttctccctccacgtaaagcagaaaatgccagatctcccttgccctgcttgctttgcagggaggatgtgactccacaatccaggttcccccaatctgtggccacacccaggatgaggatcagaagctagtgaccaccagcatcgctcctggtagctgatggcaacgtgagggaaactgcctcatttcacaggtaacagggtcagaagttctgttggcagccaacacagttcccagaccagctctgtgttccaatgtgacttgggttcatttatgtggctaactcaacttccctgtcctttccagaggttccatgagctcttcttttaaacatgtactgggcacttataggctctcatttcctgagctcgggactaaaccctctacacatccagcattcctttactaagcccctttgcccccagagctaggaggtgtggctcacaggcagggatcatcctctgctttcctccaaggcctggaccagaaggaccaagggaagacagttccagcccagagccatttcccttccaacctcttggcaagcctgatgagttccactccccgctgacgggcacacctgccttccaggcactgatcctgctttccccctcttgctctgccactcactgtgcctggcttgctgcccagccctccccagccttctctcctcctacctttcccacttattgcctccttccaggcttgtccagcatgataaactctggtctcagcattcacagcctcctctatctctcagctgtgtccctggtcatgactctgcttgctcttccctaaagcaattaaaataggaaaatctgacccttctcacccaggaggcaggtcctctcctatccactggagacccagagcaaaagctctctcctcccttcatcctccttctcaccatgtgatttcagacaagtcctttcacttccgagttttgccatgtgtgcctgtgtgcatatgtatgtgatgtacagacctctggagccatttcaccacagtgcctctccactcccagccagtgccagggcaccccctcagctgctgcaggatgtgtcaccagaaggagagagttaaaggggaagaaagcccttgagtaggagccaagtcatctgaacgcacaccctgtgcccagaggaggaggggcaagagttgctttccatgaagagtgcacctgatgagaaggcagctccagaggactcaaaggaaaaccaagaatcaagagagaaagaaacgtgcagtccttgcctacttggggagggggaggggtcgtaccacaaactccttggtcaatatagggacctgcttctccgtgcgccccagccccctctgcaccatgcactctcctcccgggcctagcgcctgctacaactgtggcctccactaatttcgggggtgcgaggcggtggatgatgcccaagtgaagccgttcaggcctcgtggcagcaccagatcaagggcgaggttgcgctgctcgtcctcagagtacacaggccggtagcccagcagctgcagcgcaccagcgcacagttcctgcacgcggcggatcttggcaaagggcagcgcatggcgccaggcctgggagacgttgagcgcattcctggacgaagtcttgaaggcttcgcggcgcgcaccaggtccagatccgtgggtgatgttatggatccaggcctcgagctgtggcgtgagactgagcccagtgaaggcgtagagcgcacggatttctgccagcggctcccgcgccaggtcctcgaagcgcaccaggcggtagcggccgcgcagaaagggtggcggcttgagtgtggcggcctcggcgatgcgtacgtggctacggcacacctcgcgcaccacgcgcaggccggggtcggcctccacccacgtgccgttggtgcccagcacgatgccgttgtcacgcgccagagccttggctgtctgctcccgggagcgcagcacggcccgcgggtcgcgcaccaggtgcacgatgcgtaggttgagcgcggggtcgctgagcagcgggtagagcacctgcaggttgaagaagcgcacctccttgagcaccacgtggctgtaggagcggcaggcctcccgggccagggtgaaggactgccgcgcgcacagtggcttgcacacggcctcgctgctgatggcgcctcggggaaaggcactgcaggcgggtggcgagcacagtgcacggctcacggcccactggaagaggtcggacaggttgcggcgccaaggcagataggcatcaaacacgtccatgtcgcacaggaagacggagcgcaccaggtcgcgcacagccatgtgcagcgttgcggcgctgccctgcgacagggtggtccacacgtgccacgcgggctccattaggtagaagacgtcggggtgctggttgaagagttggcccacgaaggacgagcccgagcgccacgaggacagcaccagcacatgcacgcgcgcctcgccgcctgctggggacgagggccctggccgggaaaccagaaagaggaggaggaaggtctgcgccaggaggagcgcggtcactgctgtgctggagacgcgcggcagccacatgctgactgctgggggccactgtccagggctgctgggagagctgcaacgctgatcacaaatccatgggagatgattagaggttcctcagcacccatggacccctcagctgagggaagcattcactttctgcttaagtccttgggagatgagtttctgtcacttacacccaagagtggtgattagatagtgacagtgaaacccttggtggggtgaggtgggaagggtgcaggggcagagcttctgggggctggccctgcgttgtttctctctgacagtgctaattacatgggtgtgttcagtttgtgaaagttcaccaagctgtactttcattatatgtactctgaagaatggcatacttcaataaaaagtaaagaatcctgactgaagaagatagtaagagtcatgtcaaggaatgtcccaaacaacaaatgagtagaggacatgaacaaatacttgccattgcactcagatactctgtggtccacatccagagggaggaattccccagtagcccacatggctttctgccgagcaccttaaagtcacaggatcttctaaacatcccttaccatttcttggcctggcctgagagacctaggaaggagctatggttctgcctgatttgcaaataggaaaagcaagacattgaccaaggatggttttccatagcagggttgagctggagcccaggagtcctggctctctgggcagcactcacttccagccaagctctgcctaccctcgacacagcagctccaggccgggagtggtggctcacacctgtaataccagcat

SEQ ID NO: 15227 - RNA, 3413 nt, Homo sapiens
  source 1..3413: mol_type = other RNA
gctgggattacaggcatgagccactgcatccagccaagttacccactcttaaggtattttgttataaccacctgaacaagaacaaagacattctctaagccatgtagtacacattcataaatctggggttttaaataccttcctcctataattgtcacgagggacagattcaagtttcatttggttgaagcttctaaacctggaaggaacctaaaatgagcttcagcttcaaggctaatgtgcctgttctccctccacgtaaagcagaaaatgccagatctcccttgccctgcttgctttgcagggaggatgtgactccacaatccaggttcccccaatctgtggccacacccaggatgaggatcagaagctagtgaccaccagcatcgctcctggtagctgatggcaacgtgagggaaactgcctcatttcacaggtaacagggtcagaagttctgttggcagccaacacagttcccagaccagctctgtgttccaatgtgacttgggttcatttatgtggctaactcaacttccctgtcctttccagaggttccatgagctcttcttttaaacatgtactgggcacttataggctctcatttcctgagctcgggactaaaccctctacacatccagcattcctttactaagcccctttgcccccagagctaggaggtgtggctcacaggcagggatcatcctctgctttcctccaaggcctggaccagaaggaccaagggaagacagttccagcccagagccatttcccttccaacctcttggcaagcctgatgagttccactccccgctgacgggcacacctgccttccaggcactgatcctgctttccccctcttgctctgccactcactgtgcctggcttgctgcccagccctccccagccttctctcctcctacctttcccacttattgcctccttccaggcttgtccagcatgataaactctggtctcagcattcacagcctcctctatctctcagctgtgtccctggtcatgactctgcttgctcttccctaaagcaattaaaataggaaaatctgacccttctcacccaggaggcaggtcctctcctatccactggagacccagagcaaaagctctctcctcccttcatcctccttctcaccatgtgatttcagacaagtcctttcacttccgagttttgccatgtgtgcctgtgtgcatatgtatgtgatgtacagacctctggagccatttcaccacagtgcctctccactcccagccagtgccagggcaccccctcagctgctgcaggatgtgtcaccagaaggagagagttaaaggggaagaaagcccttgagtaggagccaagtcatctgaacgcacaccctgtgcccagaggaggaggggcaagagttgctttccatgaagagtgcacctgatgagaaggcagctccagaggactcaaaggaaaaccaagaatcaagagagaaagaaacgtgcagtccttgcctacttggggagggggaggggtcgtaccacaaactccttggtcaatatagggacctgcttctccgtgcgccccagccccctctgcaccatgcactctcctcccgggcctagcgcctgctacaactgtggcctccactaatttcgggggtgcgaggcggtggatgatgcccaagtgaagccgttcaggcctcgtggcagcaccagatcaagggcgaggttgcgctgctcgtcctcagagtacacaggccggtagcccagcagctgcagcgcaccagcgcacagttcctgcacgcggcggatcttggcaaagggcagcgcatggcgccaggcctgggagacgttgagcgcattcctggacgaagtcttgaaggcttcgcggcgcgcaccaggtccagatccgtgggtgatgttatggatccaggcctcgagctgtggcgtgagactgagcccagtgaaggcgtagagcgcacggatttctgccagcggctcccgcgccaggtcctcgaagcgcaccaggcggtagcggccgcgcagaaagggtggcggcttgagtgtggcggcctcggcgatgcgtacgtggctacggcacacctcgcgcaccacgcgcaggccggggtcggcctccacccacgtgccgttggtgcccagcacgatgccgttgtcacgcgccagagccttggctgtctgctcccgggagcgcagcacggcccgcgggtcgcgcaccaggtgcacgatgcgtaggttgagcgcggggtcgctgagcagcgggtagagcacctgcaggttgaagaagcgcacctccttgagcaccacgtggctgtaggagcggcaggcctcccgggccagggtgaaggactgccgcgcgcacagtggcttgcacacggcctcgctgctgatggcgcctcggggaaaggcactgcaggcgggtggcgagcacagtgcacggctcacggcccactggaagaggtcggacaggttgcggcgccaaggcagataggcatcaaacacgtccatgtcgcacaggaagacggagcgcaccaggtcgcgcacagccatgtgcagcgttgcggcgctgccctgcgacagggtggtccacacgtgccacgcgggctccattaggtagaagacgtcggggtgctggttgaagagttggcccacgaaggacgagcccgagcgccacgaggacagcaccagcacatgcacgcgcgcctcgccgcctgctggggacgagggccctggccgggaaaccagaaagaggaggaggaaggtctgcgccaggaggagcgcggtcactgctgtgctggagacgcgcggcagccacatgctgactgctgggggccactgtccagggctgctgggagagctgcaacgctgatcacaaatccatgggagatgattagaggttcctcagcaccccaaagcttggcggctctgcccgagctgcagcggcacggtgggggacgcctctctccctggactcagcaaaggctcccaaacgtcgtctcttccaaattccaccgcacagccagctctttctcttcactgggagggtccgcaggggctgacttgctccttaaggtcccaagactattaagcgacacccggtgaggccgggaaaggggctctaagaggcatggacgagagttggcggtgaccaagccactggaagctcctggagactcgaggtagaacgaatgtgggaacagggcaggagtcccagaatgggatgttgaggctgggggtgtcctggggctaccacagggaaggacccggcgcagagctccctctggaacccggcactgcggcccgcgccctctactccccgcgcgccggccggcaaccctcggcgctgcccggtgcagcccgcccgagcgcacacaatgaggcgctttcagacgtggctgcggtcccgaggt

SEQ ID NO: 15228 - RNA, 3726 nt, Homo sapiens
  source 1..3726: mol_type = other RNA
gctgggattacaggcatgagccactgcatccagccacagattcattcattcattcgttctttctttgttttaagactagtcaagtgcagtagtgagaagaggggaagagtagaacaaggagcttgatctataactgactgcgaacaatcaattgagctaactcactaccttcagaccagccacaaattcatttctttagaaaaaagatgagaattattttctaaaaactgagcaatggaaaaggaaccccttcaatgggtaaagggaggtaaagttaactgaatggccttattcatcatacacattcaagttttatcacagttgtaaggtctggtaaatttttgagtagtgcttctcaagcaaggggagtggggagaggtacatcccattaggaatgtgccaccctccccaccatagtcttttttgagacaatgccatggtgagcaattgttaccaatgggaatgtgtcacatgtcttaaatgtagtgagacactttttaaaaattaagacccactccagtgaggtcttcagctgaccccctgccaaccttttagactttctgagatggcttggatgaaattatactcacattagacatctaatgcctattatttaatacttaatgataattaatatatttgaaccccttctcattttgcataggaagctttcaaatcagtgttctgcaaactgtcgtaaaattctgatttataacactgtccccaaaagtatataatgggactaaagtttaccaaacttataaaaatgttatgaaacactggatcttattttgttgatttaacatttcatttccatcattaagcatgtgaaaaagcaacataagcaaagattaaataatctaaaaatccttcaaattggtcactcattatttcagtacttactgagctaaacattattttgttacctataaaggagagaatgtaaaacactgtatgtctttggcattactagaaaggggtatttaaactttgtacctttttttgccataaaattgaagttacagtaagatgaaatggaagctcacaagccctgttggtgtggaattccactaataatgtcagattgttgccagaaaaacaaattttgtcatgcagcttgcaattaatgtaccaaaaatttaccagcccatataattttatcagtctgccttccccagaggaagtaaacagataataaaactaacgaaatcatatttcttgaccactctcatccaatataaattgttacttgtccttcgagtattagacagtgagctgtttacaaggccattcaaatgtctgggctagttaatggtagaggcagtagtctaaaatatggagtattcctgagtcagcaaagaggatcctgcattgtgaggaagcccccctaagtcattaccaagtgcagatctgggtttgatgggcctctgtcaaaagttgttttgcatccgcatttctgtgttccctgaaaacaccatgaaatactgaactttaatcagtaatgcaacaaatgagaaaatgctcagtgttttagaactattcagagtagaaaacgctggaacataaaatgaggttacgccttagttggtgagttgctaaaacttgagatcaggcgaaacaaagctgataggtctaatgccttttggaacatgtaacaccagcagttcttcaagtttggcctctggccctcctgtattagaatcatctgggagacttgctccagtgcagatctcctctacaaaacctacatttaacctagtgaagcagaaccccctggttttccctaggagtctgcatttgtcacaagcttactggatgtttctgattcacagtaaagcttgagaacactatatgtgaccaccccactggcaaggtgattaacttcttatgcatatggatactaaattttgcaacatatttgaaatgctgaagcaatatcaaatgtatgacatccccaaatatagcaatttccattggtttaaaaggtggcatatgagcacaaccaattgggattaactcagtcaactcttatggtttaacacattttacctgcactgaaaaatactttgcagatcaaactggcaaccagaaaacagaacataacagaacacatgacaccccgctgtggacttttaagaaaaaaactgacaaactccaaatccataatgacatgagaacttacactttgaaggcagaatggacttgtgggaagagaggactccccttctgttctcccttcactaggtggagaagggaagaagggctctccccagacagctctcttcattctggaatgttttgccagtccccaaggcactcagtgaccaactttctttcacaggtcctcccagtgactgacctggctcattctccgaaagtggttgacaggccactacgagagctcttgagagaagctttgtgacatgaaattcatcaaatgaagcaagattcatttttaaagaataatacaaagctccagagtaatatgcttaatccaaatgtttaaatagaatttaaaaccacattttaagtaaatttaaaattaatgaaatatcaatagtttgccttaacaaggacttgcttgaaccatattctccttttaaaatcacacacacagaatcagtgtacatttagagaaatttccccagctgaataacatttttgacatgaattcattcaaaagacaccaaccattatgaatattttaggccatgataagctgtaaccacctccggcttatggtggttaggatgttgcagcttaatgttgacatctggcatgaaaagcttatggtctgagtcatgtttcttttttatgtaattctggcttgggaatccgatacagagcagctgagaaataaattatgttgctgaggctgaagatgatgcacagaagtatggctccagctatctgagagaaagagaagggcttggaggtggccaggagccattccttcctcagagtcttgtccagaagtatggcttccatctgcatgtgcgtggccaggatcacacacacgtgaaacagctggtgactgtgaccgatgtagtcaaagcgtccaggggctaggcgttctggcagatgtgcagagtacaagaaagaggccaggagggtcatgatcatgtgcttctggtggtacgaggtggcttcattttgtgcactctcccctgggaacaggaatagcctgtagaagatggggagggagtcccaggtgtacggataagcaaaggcgaggacacgaatcaccttacagagtctgggcttctggatttcaagaaaccagaagggcagcaagtgagtccaaatgttgagagtctcattggtcatttggaaaaggctgaggatgcaggcagtggcagaactctgtggatggcggtagccgaacaggatgccttgctcatggaacaccacaggtcaggaaccttgtacaggaactctgtgtggacaaggtatgaggccagattccccaaagggctttaattggctctaaaagtcaactttcatctttaaaggaagcatgccattccagtcaaatccttggtaaaatgcccagtttctccaatggtgtcctgggttccaagggtctcgggagtccagtggacagggcgcggggacagcacaggcaggccggagaccagacactcctcccgggctgcggcgaccccggactcgcgggccctgcacctggccctgcgggtcgccgcgcctacccatgccggtccccgc

SEQ ID NO: 15229 - RNA, 3868 nt, Homo sapiens
  source 1..3868: mol_type = other RNA
gctgggattacaggcatgagccactgcatccagccacagattcattcattcattcgttctttctttgttttaagactagtcaagtgcagtagtgagaagaggggaagagtagaacaaggagcttgatctataactgactgcgaacaatcaattgagctaactcactaccttcagaccagccacaaattcatttctttagaaaaaagatgagaattattttctaaaaactgagcaatggaaaaggaaccccttcaatgggtaaagggaggtaaagttaactgaatggccttattcatcatacacattcaagttttatcacagttgtaaggtctggtaaatttttgagtagtgcttctcaagcaaggggagtggggagaggtacatcccattaggaatgtgccaccctccccaccatagtcttttttgagacaatgccatggtgagcaattgttaccaatgggaatgtgtcacatgtcttaaatgtagtgagacactttttaaaaattaagacccactccagtgaggtcttcagctgaccccctgccaaccttttagactttctgagatggcttggatgaaattatactcacattagacatctaatgcctattatttaatacttaatgataattaatatatttgaaccccttctcattttgcataggaagctttcaaatcagtgttctgcaaactgtcgtaaaattctgatttataacactgtccccaaaagtatataatgggactaaagtttaccaaacttataaaaatgttatgaaacactggatcttattttgttgatttaacatttcatttccatcattaagcatgtgaaaaagcaacataagcaaagattaaataatctaaaaatccttcaaattggtcactcattatttcagtacttactgagctaaacattattttgttacctataaaggagagaatgtaaaacactgtatgtctttggcattactagaaaggggtatttaaactttgtacctttttttgccataaaattgaagttacagtaagatgaaatggaagctcacaagccctgttggtgtggaattccactaataatgtcagattgttgccagaaaaacaaattttgtcatgcagcttgcaattaatgtaccaaaaatttaccagcccatataattttatcagtctgccttccccagaggaagtaaacagataataaaactaacgaaatcatatttcttgaccactctcatccaatataaattgttacttgtccttcgagtattagacagtgagctgtttacaaggccattcaaatgtctgggctagttaatggtagaggcagtagtctaaaatatggagtattcctgagtcagcaaagaggatcctgcattgtgaggaagcccccctaagtcattaccaagtgcagatctgggtttgatgggcctctgtcaaaagttgttttgcatccgcatttctgtgttccctgaaaacaccatgaaatactgaactttaatcagtaatgcaacaaatgagaaaatgctcagtgttttagaactattcagagtagaaaacgctggaacataaaatgaggttacgccttagttggtgagttgctaaaacttgagatcaggcgaaacaaagctgataggtctaatgccttttggaacatgtaacaccagcagttcttcaagtttggcctctggccctcctgtattagaatcatctgggagacttgctccagtgcagatctcctctacaaaacctacatttaacctagtgaagcagaaccccctggttttccctaggagtctgcatttgtcacaagcttactggatgtttctgattcacagtaaagcttgagaacactatatgtgaccaccccactggcaaggtgattaacttcttatgcatatggatactaaattttgcaacatatttgaaatgctgaagcaatatcaaatgtatgacatccccaaatatagcaatttccattggtttaaaaggtggcatatgagcacaaccaattgggattaactcagtcaactcttatggtttaacacattttacctgcactgaaaaatactttgcagatcaaactggcaaccagaaaacagaacataacagaacacatgacaccccgctgtggacttttaagaaaaaaactgacaaactccaaatccataatgacatgagaacttacactttgaaggcagaatggacttgtgggaagagaggactccccttctgttctcccttcactaggtggagaagggaagaagggctctccccagacagctctcttcattctggaatgttttgccagtccccaaggcactcagtgaccaactttctttcacaggtcctcccagtgactgacctggctcattctccgaaagtggttgacaggccactacgagagctcttgagagaagctttgtgacatgaaattcatcaaatgaagcaagattcatttttaaagaataatacaaagctccagagtaatatgcttaatccaaatgtttaaatagaatttaaaaccacattttaagtaaatttaaaattaatgaaatatcaatagtttgccttaacaaggacttgcttgaaccatattctccttttaaaatcacacacacagaatcagtgtacatttagagaaatttccccagctgaataacatttttgacatgaattcattcaaaagacaccaaccattatgaatattttaggccatgataagctgtaaccacctccggcttatggtggttaggatgttgcagcttaatgttgacatctggcatgaaaagcttatggtctgagtcatgtttcttttttatgtaattctggcttgggaatccgatacagagcagctgagaaataaattatgttgctgaggctgaagatgatgcacagaagtatggctccagctatctgagagaaagagaagggcttggaggtggccaggagccattccttcctcagagtcttgtccagaagtatggcttccatctgcatgtgcgtggccaggatcacacacacgtgaaacagctggtgactgtgaccgatgtagtcaaagcgtccaggggctaggcgttctggcagatgtgcagagtacaagaaagaggccaggagggtcatgatcatgtgcttctggtggtacgaggtggcttcattttgtgcactctcccctgggaacaggaatagcctgtagaagatggggagggagtcccaggtgtacggataagcaaaggcgaggacacgaatcaccttacagagtctgggcttctggatttcaagaaaccagaagggcagcaagtgagtccaaatgttgagagtctcattggtcatttggaaaaggctgaggatgcaggcagtggcagaactctgtggatggcggtagccgaacaggatgccttgctcatggaacacctggggtatctggtctatgctaaacagcctggggagcttcaggctcagcatcttggagctggattggcaaggccagtaggtgacagcgcctccctgttaccaggcctcactcaaagctctaacatggcctggggcgtctctgcctagctggtgctgtgccgcttcccacaggtcaggaaccttgtacaggaactctgtgtggacaaggtatgaggccagattccccaaagggctttaattggctctaaaagtcaactttcatctttaaaggaagcatgccattccagtcaaatccttggtaaaatgcccagtttctccaatggtgtcctgggttccaagggtctcgggagtccagtggacagggcgcggggacagcacaggcaggccggagaccagacactcctcccgggctgcggcgaccccggactcgcgggccctgcacctggccctgcgggtcgcc

SEQ ID NO: 15230 - RNA, 4213 nt, Homo sapiens
  source 1..4213: mol_type = other RNA
gctgggattacaggcatgagccactgcatccagccacagattcattcattcattcgttctttctttgttttaagactagtcaagtgcagtagtgagaagaggggaagagtagaacaaggagcttgatctataactgactgcgaacaatcaattgagctaactcactaccttcagaccagccacaaattcatttctttagaaaaaagatgagaattattttctaaaaactgagcaatggaaaaggaaccccttcaatgggtaaagggaggtaaagttaactgaatggccttattcatcatacacattcaagttttatcacagttgtaaggtctggtaaatttttgagtagtgcttctcaagcaaggggagtggggagaggtacatcccattaggaatgtgccaccctccccaccatagtcttttttgagacaatgccatggtgagcaattgttaccaatgggaatgtgtcacatgtcttaaatgtagtgagacactttttaaaaattaagacccactccagtgaggtcttcagctgaccccctgccaaccttttagactttctgagatggcttggatgaaattatactcacattagacatctaatgcctattatttaatacttaatgataattaatatatttgaaccccttctcattttgcataggaagctttcaaatcagtgttctgcaaactgtcgtaaaattctgatttataacactgtccccaaaagtatataatgggactaaagtttaccaaacttataaaaatgttatgaaacactggatcttattttgttgatttaacatttcatttccatcattaagcatgtgaaaaagcaacataagcaaagattaaataatctaaaaatccttcaaattggtcactcattatttcagtacttactgagctaaacattattttgttacctataaaggagagaatgtaaaacactgtatgtctttggcattactagaaaggggtatttaaactttgtacctttttttgccataaaattgaagttacagtaagatgaaatggaagctcacaagccctgttggtgtggaattccactaataatgtcagattgttgccagaaaaacaaattttgtcatgcagcttgcaattaatgtaccaaaaatttaccagcccatataattttatcagtctgccttccccagaggaagtaaacagataataaaactaacgaaatcatatttcttgaccactctcatccaatataaattgttacttgtccttcgagtattagacagtgagctgtttacaaggccattcaaatgtctgggctagttaatggtagaggcagtagtctaaaatatggagtattcctgagtcagcaaagaggatcctgcattgtgaggaagcccccctaagtcattaccaagtgcagatctgggtttgatgggcctctgtcaaaagttgttttgcatccgcatttctgtgttccctgaaaacaccatgaaatactgaactttaatcagtaatgcaacaaatgagaaaatgctcagtgttttagaactattcagagtagaaaacgctggaacataaaatgaggttacgccttagttggtgagttgctaaaacttgagatcaggcgaaacaaagctgataggtctaatgccttttggaacatgtaacaccagcagttcttcaagtttggcctctggccctcctgtattagaatcatctgggagacttgctccagtgcagatctcctctacaaaacctacatttaacctagtgaagcagaaccccctggttttccctaggagtctgcatttgtcacaagcttactggatgtttctgattcacagtaaagcttgagaacactatatgtgaccaccccactggcaaggtgattaacttcttatgcatatggatactaaattttgcaacatatttgaaatgctgaagcaatatcaaatgtatgacatccccaaatatagcaatttccattggtttaaaaggtggcatatgagcacaaccaattgggattaactcagtcaactcttatggtttaacacattttacctgcactgaaaaatactttgcagatcaaactggcaaccagaaaacagaacataacagaacacatgacaccccgctgtggacttttaagaaaaaaactgacaaactccaaatccataatgacatgagaacttacactttgaaggcagaatggacttgtgggaagagaggactccccttctgttctcccttcactaggtggagaagggaagaagggctctccccagacagctctcttcattctggaatgttttgccagtccccaaggcactcagtgaccaactttctttcacaggtcctcccagtgactgacctggctcattctccgaaagtggttgacaggccactacgagagctcttgagagaagctttgtgacatgaaattcatcaaatgaagcaagattcatttttaaagaataatacaaagctccagagtaatatgcttaatccaaatgtttaaatagaatttaaaaccacattttaagtaaatttaaaattaatgaaatatcaatagtttgccttaacaaggacttgcttgaaccatattctccttttaaaatcacacacacagaatcagtgtacatttagagaaatttccccagctgaataacatttttgacatgaattcattcaaaagacaccaaccattatgaatattttaggccatgataagctgtaaccacctccggcttatggtggttaggatgttgcagcttaatgttgacatctggcatgaaaagcttatggtctgagtcatgtttcttttttatgtaattctggcttgggaatccgatacagagcagctgagaaataaattatgttgctgaggctgaagatgatgcacagaagtatggctccagctatctgagagaaagagaagggcttggaggtggccaggagccattccttcctcagagtcttgtccagaagtatggcttccatctgcatgtgcgtggccaggatcacacacacgtgaaacagctggtgactgtgaccgatgtagtcaaagcgtccaggggctaggcgttctggcagatgtgcagagtacaagaaagaggccaggagggtcatgatcatgtgcttctggtggtacgaggtggcttcattttgtgcactctcccctgggaacaggaatagcctgtagaagatggggagggagtcccaggtgtacggataagcaaaggcgaggacacgaatcaccttacagagtctgggcttctggatttcaagaaacctggagtagcaggagaggcctgtgctgaggatggtgttcagtacagccagggccacgtagtagtcatggaaagtggtgcacatgagcgcatccgggaacgtgtatgcagagtaggcaatggctgagcccaggctgaagaggttgacggcaccatagtccaggaagtagcaaatgtgccgggcattcttggacatagagctgaaggtgtgcgcacagctggacacaagtgggtacacgcagctggtgcacatgtacacaagcatgggccaggagtagctgtcattcttgatgtctgtcatatacagtgcagtcacaaacctccatgcaaagaaccagaagggcagcaagtgagtccaaatgttgagagtctcattggtcatttggaaaaggctgaggatgcaggcagtggcagaactctgtggatggcggtagccgaacaggatgccttgctcatggaacacctggggtatctggtctatgctaaacagcctggggagcttcaggctcagcatcttggagctggattggcaaggccagtaggtgacagcgcctccctgttaccaggcctcactcaaagctctaacatggcctggggcgtctctgcctagctggtgctgtgccgcttcccacaggtcaggaaccttgtacaggaactctgtgtggacaaggtatgaggccagattccccaaagggctttaattggctctaaaagtcaactttcatctttaaaggaagcatgccattccagtcaaatccttggtaaaatgcccagtttctccaatggtgtcctgggttccaagggtctcgggagtccagtggacagggcgcggggacagcacaggcaggccggagaccagacactcctcccgggctgcggcgaccccggactcgcgggccctgcacctggccctgcgggtcgccgcgcctacccat

SEQ ID NO: 15231 - RNA, 4460 nt, Homo sapiens
  source 1..4460: mol_type = other RNA
gctgggattacaggcatgagccactgcatccagccacagattcattcattcattcgttctttctttgttttaagactagtcaagtgcagtagtgagaagaggggaagagtagaacaaggagcttgatctataactgactgcgaacaatcaattgagctaactcactaccttcagaccagccacaaattcatttctttagaaaaaagatgagaattattttctaaaaactgagcaatggaaaaggaaccccttcaatgggtaaagggaggtaaagttaactgaatggccttattcatcatacacattcaagttttatcacagttgtaaggtctggtaaatttttgagtagtgcttctcaagcaaggggagtggggagaggtacatcccattaggaatgtgccaccctccccaccatagtcttttttgagacaatgccatggtgagcaattgttaccaatgggaatgtgtcacatgtcttaaatgtagtgagacactttttaaaaattaagacccactccagtgaggtcttcagctgaccccctgccaaccttttagactttctgagatggcttggatgaaattatactcacattagacatctaatgcctattatttaatacttaatgataattaatatatttgaaccccttctcattttgcataggaagctttcaaatcagtgttctgcaaactgtcgtaaaattctgatttataacactgtccccaaaagtatataatgggactaaagtttaccaaacttataaaaatgttatgaaacactggatcttattttgttgatttaacatttcatttccatcattaagcatgtgaaaaagcaacataagcaaagattaaataatctaaaaatccttcaaattggtcactcattatttcagtacttactgagctaaacattattttgttacctataaaggagagaatgtaaaacactgtatgtctttggcattactagaaaggggtatttaaactttgtacctttttttgccataaaattgaagttacagtaagatgaaatggaagctcacaagccctgttggtgtggaattccactaataatgtcagattgttgccagaaaaacaaattttgtcatgcagcttgcaattaatgtaccaaaaatttaccagcccatataattttatcagtctgccttccccagaggaagtaaacagataataaaactaacgaaatcatatttcttgaccactctcatccaatataaattgttacttgtccttcgagtattagacagtgagctgtttacaaggccattcaaatgtctgggctagttaatggtagaggcagtagtctaaaatatggagtattcctgagtcagcaaagaggatcctgcattgtgaggaagcccccctaagtcattaccaagtgcagatctgggtttgatgggcctctgtcaaaagttgttttgcatccgcatttctgtgttccctgaaaacaccatgaaatactgaactttaatcagtaatgcaacaaatgagaaaatgctcagtgttttagaactattcagagtagaaaacgctggaacataaaatgaggttacgccttagttggtgagttgctaaaacttgagatcaggcgaaacaaagctgataggtctaatgccttttggaacatgtaacaccagcagttcttcaagtttggcctctggccctcctgtattagaatcatctgggagacttgctccagtgcagatctcctctacaaaacctacatttaacctagtgaagcagaaccccctggttttccctaggagtctgcatttgtcacaagcttactggatgtttctgattcacagtaaagcttgagaacactatatgtgaccaccccactggcaaggtgattaacttcttatgcatatggatactaaattttgcaacatatttgaaatgctgaagcaatatcaaatgtatgacatccccaaatatagcaatttccattggtttaaaaggtggcatatgagcacaaccaattgggattaactcagtcaactcttatggtttaacacattttacctgcactgaaaaatactttgcagatcaaactggcaaccagaaaacagaacataacagaacacatgacaccccgctgtggacttttaagaaaaaaactgacaaactccaaatccataatgacatgagaacttacactttgaaggcagaatggacttgtgggaagagaggactccccttctgttctcccttcactaggtggagaagggaagaagggctctccccagacagctctcttcattctggaatgttttgccagtccccaaggcactcagtgaccaactttctttcacaggtcctcccagtgactgacctggctcattctccgaaagtggttgacaggccactacgagagctcttgagagaagctttgtgacatgaaattcatcaaatgaagcaagattcatttttaaagaataatacaaagctccagagtaatatgcttaatccaaatgtttaaatagaatttaaaaccacattttaagtaaatttaaaattaatgaaatatcaatagtttgccttaacaaggacttgcttgaaccatattctccttttaaaatcacacacacagaatcagtgtacatttagagaaatttccccagctgaataacatttttgacatgaattcattcaaaagacaccaaccattatgaatattttaggccatgataagctgtaaccacctccggcttatggtggttaggatgttgcagcttaatgttgacatctggcatgaaaagcttatggtctgagtcatgtttcttttttatgtaattctggcttgggaatccgatacagagcagctgagaaataaattatgttgctgaggctgaagatgatgcacagaagtatggctccagctatctgagagaaagagaagggcttggaggtggccaggagccattccttcctcagagtcttgtccagaagtatggcttccatctgcatgtgcgtggccaggatcacacacacgtgaaacagctggtgactgtgaccgatgtagtcaaagcgtccaggggctaggcgttctggcagatgtgcagagtacaagaaagaggccaggagggtcatgatcatgtgcttctggtggtacgaggtggcttcattttgtgcactctcccctgggaacaggaatagcctgtagaagatggggagggagtcccaggtgtacggataagcaaaggcgaggacacgaatcaccttacagagtctgggcttctggatttcaagaaacctggagtagcaggagaggcctgtgctgaggatggtgttcagtacagccagggccacgtagtagtcatggaaagtggtgcacatgagcgcatccgggaacgtgtatgcagagtaggcaatggctgagcccaggctgaagaggttgacggcaccatagtccaggaagtagcaaatgtgccgggcattcttggacatagagctgaaggtgtgcgcacagctggacacaagtgggtacacgcagctggtgcacatgtacacaagcatgggccaggagtagctgtcattcttgatgtctgtcatatacagtgcagtcacaaacctccatgcaaagaaccagaagggcagcaagtgagtccaaatgttgagagtctcattggtcatttggaaaaggctgaggatgcaggcagtggcagaactctgtggatggcggtagccgaacaggatgccttgctcatggaacacctggggtatctggtctatgctaaacagcctggggagcttcaggctcagcatcttggagctggattggcaaggccagtaggtgacagcgcctccctgttaccaggcctcactcaaagctctaacatggcctggggcgtctctgcctagctggtgctgtgccgcttcccacaggtcaggaaccttgtacaggaactctgtgtggacaaggtatgaggccagattccccaaagggctttaattggctctaaaagtcaactttcatctttaaaggaagcatgccattccagtcaaatccttggtaaaatgcccagtttctccaatggtgtcctttatcaggagagctgttttccctttgaaagtcaaatctgaggccttgggacaatgcggggtgttcccagcacaccaggcccggtggaggaggcccagccagaggctccctctcctccccagcacactgcccagccagcctgcaagagcacggctggaattcacctcctcagactcctcctctgttcttttcaggcctttaaggtaatcctgagggtgtgaagcaaagactttatcatccatgggggggaatggtccagatacctaaaggcaaaaatgatgcatccagaagaaaggccaggtaggaatccaaggcccagagatgttgggtggctgctcaggaccacacagcgagctgatcgcgggtccagaggccatggtcttgttaagct

SEQ ID NO: 15232 - RNA, 3666 nt, Homo sapiens
  source 1..3666: mol_type = other RNA
gctgggattacaggcatgagccactgcatccagcttgcttctaattttcctacccaggctgttttaaacctagttctccagctaagtaaaatgtgcccaaatggaaaacatctaaatcttctgcagcccattcttcctgtgtctttgtgttgacaaacctctaatcttccatgtctttgtgttgacaaacctaaccttccatgtctttttgttgacaaacctctaaccttccatgtctttgtgttgacaaacctctccatgggtggtgcatctgaccctatcccaacatgccttaggacgctcatctccttgactgtctgccatcccctcccaaaactaagtggaggctctgtcttttcctcctagtttgaggttctcttctcccagtgtctaaaatgatcaatatgcctagagtagatgctgctgaagaggcaaagtagtaatcctgccacctggaagcaaaggctgtgggttggagggggaagcgggtgtgagggctgatgataagccctaggaggctcctgagtcatattcctatgtttgctctctggagagatgggctaaactgtttatcttttaaaaaccagatgattaaaaagttacattttagtattatactgataggaatataggataatctcttctaaagcctatttggtttccagaagagttagatacttgaacaagagtggacagagtaagatacctagctacagcaatagaaatcacaaactgttctgtggttttaatcttcctatttctgatttagaagtatgaagtgatcatatttaatctttctgctcctgctcaaaaataattctataacatcatttaggttatagaaagtttctacttatagcccttacattctttatgaccgaaatctgtgtctttcctcatgactgataattatctcccaatttggtcacttctgctaattgctattttattaaacttgaaattttaggttgggaagcaaagggaaaccactgggcatcccctttgtttctagggagaaaagactaacttgtcccatctgctcacttgcttatggagctaaaagacccccagtcctagaagtgttctgttcctgaggagtggttaaagaggtgaaaagaagaggtgaattaaaagatgaaagagctttttaaatagccagcaactctctctaccatctgttttggtaagagctagcacctcttgttctctttagaccctggagggaataaaccaaaatcagtggttccaggatccttcagagccaaaagaccccaataccacagtcttgacctttgccctgcctgcttctgaaactggagaatggcatctcccagcagcctaaggcagacataggtcatacctatccctgggcagcgagctgagctcccacagactgagttgtgctggatctcagaattctaagcattaatgtttccttgctgttataattcttgctcatcaggttcaactgccttatccctctgaggtttgcaaatgaggatggagaagccactgagaaatggaccagtgagctgagctcaccttttatatgagtggattttttttttttttttgaaatggagtcttgctctgtcgcccaggctggagtacaatggcgtgatctcagctcactgcaacctccacctccccggttcaagcgattctcctgcctcagcctcctgggtagctgggattacaggcgcgtgccaccacgcccggcatgagtggaattttagtgttaaatctcttcctgactctgggttcagtaggtccctcctcttctgttaccctcctggttctctctgttcaccaactacctgcatgtgccaaactagaaaaaggaaataatttacacccctgccccaacagctccttccctcctagggacttctgtgtccaccccccactttgggtcttagaactgtggctagaagataaaagggaggagtttgagtcagaggctttatgtccccaaacccaaccccctctgagtattaaactatagtggcattgtccctcaagctcccctctgccttggctccagagtcttcctcctcttcttccagactgggcagggtggctgttgttattggtgaagataggcatctagccagagctgccctgactcctttagtgagtggatgatgtcggcgaaggctgacagcaggggcttggactggtactctatgccatgcttggcacacaaggactgcaccaggggagccactttgtggtaattgtgtcgaggcatcgtgggaaaaagatggtgctcaatctggaagttgaggtgtccactgaaccagtcattgaaggcagacttgtggacattgcatgtggcctggagctgggtggaaacccagtccatgttccggtcatgatcaatgtgcatgggaatatggttcatctgtgtcacccacacaaaccagttgctttccaggaacctgactatgaagaaaaggcccaggaaggctttcagccccaatagtggcacataagtgaggaagaagcggacgtagaaggtaatcatccaggccaagtccacccacttctttcgctggataacaaaatagaaaatataccactggaagtagagaggcagcaaggctgggggcccaattaggaagaagtatttgtgctggtggttgtacggcatatattttttcttctgtttcccaagctccacagagaggatcttccccaaggcaaagaagaagggatgcatgttgatgtctgggtctttgcggaagcagttgggcttggcatggtgctggaagtgcatgtggttccaccaactggcgggggcccccttcaggtggccaatcacaaaatgatgtagcagatggttccactttgaggtgctgaagaccgacaggtgcccaaagtcatgctgcagccagccagcctgggcctgaactgcactgagcagcaccgcacagaggaggaagggcaaaaaggacgtcccaaagacccaaagggtgagccaggctgcaccatccagcagcaagatgtgcagcaggtacagcaggaagaagacatggttggccttcatgagccccatccgctccactgtggcccgcagctcccggaactcatctgtcagctctttattcttggtgggctcaaagctgggctgctctggagacagttctccaatcaggagagagttcatatacttcttcacaaggcccttgttgatgtggaaggccacaaagggatccgtggcatcctgcccggcgtagtggctgatgacccgggagccccctggatgccggcgggtgaactcgctgatgttgtacaccttacggtcgatcactagccaccgctcctcgcaccctgagcgctgggccacctcgtcccaggtgaagtagcgcggggtaggtccctgagccgcggtctcggcggccaccgggtcgggggccatagctggcctggcgacgccgcgcgccgggccagcaggggctgtcaggcgcgtgctcggggtccgcgggctccaggagtggatttgctggcgcgcgcccagagccagccgcctgcgcgccgggttttcagcaccgcagggcagaccggcgggcctcgcagcgcgcgttcccattggccgagcctcgtggcgcggggagcgagatcccgtcccccggtgggtcttgggcaactcacagctgggctgcc

SEQ ID NO: 15233 - RNA, 3394 nt, Homo sapiens
  source 1..3394: mol_type = other RNA
gctgggattacaggcatgagccactgcatccagcttgcttctaattttcctacccaggctgttttaaacctagttctccagctaagtaaaatgtgcccaaatggaaaacatctaaatcttctgcagcccattcttcctgtgtctttgtgttgacaaacctctaatcttccatgtctttgtgttgacaaacctaaccttccatgtctttttgttgacaaacctctaaccttccatgtctttgtgttgacaaacctctccatgggtggtgcatctgaccctatcccaacatgccttaggacgctcatctccttgactgtctgccatcccctcccaaaactaagtggaggctctgtcttttcctcctagtttgaggttctcttctcccagtgtctaaaatgatcaatatgcctagagtagatgctgctgaagaggcaaagtagtaatcctgccacctggaagcaaaggctgtgggttggagggggaagcgggtgtgagggctgatgataagccctaggaggctcctgagtcatattcctatgtttgctctctggagagatgggctaaactgtttatcttttaaaaaccagatgattaaaaagttacattttagtattatactgataggaatataggataatctcttctaaagcctatttggtttccagaagagttagatacttgaacaagagtggacagagtaagatacctagctacagcaatagaaatcacaaactgttctgtggttttaatcttcctatttctgatttagaagtatgaagtgatcatatttaatctttctgctcctgctcaaaaataattctataacatcatttaggttatagaaagtttctacttatagcccttacattctttatgaccgaaatctgtgtctttcctcatgactgataattatctcccaatttggtcacttctgctaattgctattttattaaacttgaaattttaggttgggaagcaaagggaaaccactgggcatcccctttgtttctagggagaaaagactaacttgtcccatctgctcacttgcttatggagctaaaagacccccagtcctagaagtgttctgttcctgaggagtggttaaagaggtgaaaagaagaggtgaattaaaagatgaaagagctttttaaatagccagcaactctctctaccatctgttttggtaagagctagcacctcttgttctctttagaccctggagggaataaaccaaaatcagtggttccaggatccttcagagccaaaagaccccaataccacagtcttgacctttgccctgcctgcttctgaaactggagaatggcatctcccagcagcctaaggcagacataggtcatacctatccctgggcagcgagctgagctcccacagactgagttgtgctggatctcagaattctaagcattaatgtttccttgctgttataattcttgctcatcaggttcaactgccttatccctctgaggtttgcaaatgaggatggagaagccactgagaaatggaccagtgagctgagctcaccttttatatgagtggattttttttttttttttgaaatggagtcttgctctgtcgcccaggctggagtacaatggcgtgatctcagctcactgcaacctccacctccccggttcaagcgattctcctgcctcagcctcctgggtagctgggattacaggcgcgtgccaccacgcccggcatgagtggaattttagtgttaaatctcttcctgactctgggttcagtaggtccctcctcttctgttaccctcctggttctctctgttcaccaactacctgcatgtgccaaactagaaaaaggaaataatttacacccctgccccaacagctccttccctcctagggacttctgtgtccaccccccactttgggtcttagaactgtggctagaagataaaagggaggagtttgagtcagaggctttatgtccccaaacccaaccccctctgagtattaaactatagtggcattgtccctcaagctcccctctgccttggctccagagtcttcctcctcttcttccagactgggcagggtggctgttgttattggtgaagataggcatctagccagagctgccctgactcctttagtgagtggatgatgtcggcgaaggctgacagcaggggcttggactggtactctatgccatgcttggcacacaaggactgcaccaggggagccactttgtggtaattgtgtcgaggcatcgtgggaaaaagatggtgctcaatctggaagttgaggtgtccactgaaccagtcattgaaggcagacttgtggacattgcatgtggcctggagctgggtggaaacccagtccatgttccggtcatgatcaatgtgcatgggaatatggttcatctgtgtcacccacacaaaccagttgctttccaggaacctgactatgaagaaaaggcccaggaaggctttcagccccaatagtggcacataagtgaggaagaagcggacgtagaaggtaatcatccaggccaagtccacccacttctttcgctggataacaaaatagaaaatataccactggaagtagagaggcagcaaggctgggggcccaattaggaagaagtatttgtgctggtggttgtacggcatatattttttcttctgtttcccaagctccacagagaggatcttccccaaggcaaagaagaagggatgcatgttgatgtctgggtctttgcggaagcagttgggcttggcatggtgctggaagtgcatgtggttccaccaactggcgggggcccccttcaggtggccaatcacaaaatgatgtagcagatggttccactttgaggtgctgaagaccgacaggtgcccaaagtcatgctgcagccagccagcctgggcctgaactgcactgagcagcaccgcacagaggaggaagggcaaaaaggacgtcccaaagacccaaagggtgagccaggctgcaccatccagcagcaagatgtgcagcaggtacagcaggaagaagacatggttggccttcatgagccccatccgctccactgtggcccgcagctcccggaactcatctgtcagctctttattcttggtgggctcaaagctgggctgctctggagacagttctccaatcaggagagagttcatatacttcttcacaaggcccttgttgatgtggaaggccacaaagggatctttgggttgtgcaaggtaaggtccatggcgataagattcacgttggcaggtccggcagccccgggccctgtaagtgatgcggcgtgtggggcgggggccggggcggagccggcggccggtggcaccacacatacggaccaatcgccgtccccgccgcggcattcccggccccaaatc

SEQ ID NO: 15234 - RNA, 4146 nt, Homo sapiens
  source 1..4146: mol_type = other RNA
gctgggattacaggcatgagccactgcatccggcctgtgggcctttcttttaatgtcttatttgaggacgtggtgcagcagccttggtgtgggtgctcgaagtccctggcctcctacctgagcctcttctgtccagaggcccagtattaccttctataggtaaaactgtcaccagttttaagacttacaataagcaaagaggaaatgccctcttctgtgctgagggctgtaccctcctacccatgggagcaccaggtcggccattctcagggttggtctcctgcggtttacagagcaccacagacctgccaaaggctttccacgtttgtgcagcaatcctcgagtgtttagagaagaggaagatatcctggctggcactctttcagttgacagagagtggtaagaaacacgctgctgaggcacaaatgcggagggccgctcttttcagaggcatcttgcaaatggttaagaacgagccctccttgaggttccttgctaagtaagtttataagctccattttagttgggacagattaagcacaaacttgtttaaagcaataagataatttactggctcactggtcaaccccaggaccaatgggcctatcatggggactgcctctctctgcaccacacccaccctcctgcaagaggtcgacccccccatcctctcccagctgctgacaggtacctgggtatcctcagctcaggctgttcgccccacactatccccacagccaggcctcccagggtacacgtcccgacccccaggggtgtccccagcactgataataggcagagatgtccagagttgcctgagccacttcttggtgttgcagacctcaggctggggcggctcctcctccgtgtggccccggatcagcacaccaggctgctgcctttcgctttttacaggtacctccacccacagggctggtcagggctgggcagtgtttcccagacccccatctcagcacctctgggtcccgccagatgggaagggttgtctgtgcctctgctccacagatgagcagtatcccttggcatcacctgctacctttccagcagtctgtagccatttgtcactatgtctttacctctagtcttctctcctacttccatgaagacgcggccatcagggaagaggccttcctgcatgttgctgtggacatgtacttgaagctggtccagctcttcgtggctggggatacaagcacagtttcacctccagctggcaggagcctggagctcaagggtcaggcaggtgcaagggccagtcccacctccaggggagctccccccagccggaggctccttctgccaaagaatgttccggcacagcatgcagactatgggggacacaccagccctgtttctgtatgtcttctaacctgtgagtttgcctgttttctctctagggcaaccccgtggaactgataacaaaagctcgtctttttctgctgcagttaatacctcggtgcccgaaaaagagcttctcacacgtggcagaggtaacgtcaagatgcccaccttgggccatgtgggggacatgagaattgacagctgcctgggccatgtgcctgcctggctggcaatacaactcgactatttctgccagagcccctcccctgtggtctgaggcctagtgggcggcatgggctgaggacctgctcctctctcacagctgctggctgatcgtggggactgcgacccagaggtgagcgccgccctccagagcagacagcaggctgcccctgacgctgacctgtcccaggagcctcatctcttctgacgggacctgccactgcacaccagcccagctcccgtgtaaataatttattacaagcataacatggagctcttgttgcactaaaaagtggattacaaatctcctcgactgctttagtggggaaaggaatcaattatttatgaactgtccggccccgagtcactcagcgtttgcgggaaaataaaccactggtcccagagcagaggaaggctacttgagccggacaccaagcccgcctccagcaccaagggcgggcagcaccctccgaccctcccatgcgggtgcacacgaagggtgaggctgacacagccactgcggagtccaggctgctagaggtgctcatcctcactgccgtcctcaggtgggttcgggcttcaccgcctggccctctgtggtcacagaggggctcggtggcccaggtggtggttccgcctccaggggcagggccttgtcctgggtctgtgtcagcgggtgcaccatggacatgtgtacattgaggttgtgggccttctcaaaccgccggccacactggtcacaggcaaagtccagctcagtctcagccttgtgtttggtcatgtggtacttgagggatgcccgctgcctgcactggaacccacagacctcacactgcaaaggcttggctcccgaatgtcgcatttggtggacgagaaggtgcttccgctgcttgaaggtttgtccacattcgtcacagatatagttccgcacctctgagaggggagagtccagtgagtccaggcccctgatgctccaacctcccggggggacgacgatgacaatgtgaaaccatcacagctgtgtggatgagcttcacgtggcgctgcaggtagcggtcgatcatgaaaaccttgttgcagccagggtgggggcagggccgctcccggacctcctcgtggtgctccttgatgtgcttcttcatgccgtcagcgcctcggtacacggccgtgcagccctggtaaggacacttgtagatggtgggaagctcctccctctcacaacgaagcttcttcttccatccgggcttgggtcccggcttcttccgaattcttggttcttcagacttcttggcttctttgctttcactcttcttaccagagactttcctttctgggtaaggctcaaaggactcgtccgaagactgggcattttgcttcttgtcattttcatcttcactcaagacgtctccctcagaaaggtcactgaactcgtcttttacccgatcatccgaggttgaagatggaagctgcttctcacccaactgccctggggccctgcaaaggggcaggcttggctgaggtgggaagcccgacctgggccccaccgcgtcgctgtccgaaggaggctgggccacatccgtgctgggcagggtcttggtctcagccccaactggggtccctgtccctctaccctgggaggtctgaggggcatccccagggttccaccctcggtgctggggcagccgtggcgccgtctctttgtcccatggccacttgactgccagcgcactgtccagcaagaaggccttgcagctggagctggtatccatggtgtagtcgtggccctggtcgcagccccacacgacctggatgacgccgcagtactcggaggacagtgtcctctgaaggtggggcagggccccgcagctggccgcatgtccatgcacccaccccaccaagccgtgcaggcactgggggctggatgtgatcagatccaccagacacgctccctcctctgcccctgttgggggctgggcaccgacctttgcacaaggcttccggcgaccagccggggaggcgttgaccctctgcaggaaggacttgagaaggctgtggcactggtagaactgggcgtggcagctcttgcagacaaacggagacaaggtggggtcctggcggacagccacaccaagcaggcgctggaagtcccgtacgagcacgcgctcctctgcggatggcctctccatgctcgctccaggcgccctctcggagatgctgcgcaggcttctcgaggaaaacttcccgtggcagaggcgacagtgacccatggcgagagcccggcctgctccgtgggagacggaggcgcggggcgggcaggcgccggcggaggccacgcggcgcgcaggtggcgggcgggctgcagaaaggggaggggggccggggtctcacgtagagaggggcctggctgccgcggttagacgcccatggcaactccgtgaggggcccttctcgccagccccgtctcaagacggcgaagaggcccggctccgtcgcgacaacccacccggactctgccgcccccgccactaacacccgtggggcccgcagtacgcgcggaggggg

SEQ ID NO: 15235 - RNA, 4061 nt, Homo sapiens
  source 1..4061: mol_type = other RNA
gctgggattacaggcatgagccactgcatccggcctgtgggcctttcttttaatgtcttatttgaggacgtggtgcagcagccttggtgtgggtgctcgaagtccctggcctcctacctgagcctcttctgtccagaggcccagtattaccttctataggtaaaactgtcaccagttttaagacttacaataagcaaagaggaaatgccctcttctgtgctgagggctgtaccctcctacccatgggagcaccaggtcggccattctcagggttggtctcctgcggtttacagagcaccacagacctgccaaaggctttccacgtttgtgcagcaatcctcgagtgtttagagaagaggaagatatcctggctggcactctttcagttgacagagagtggtaagaaacacgctgctgaggcacaaatgcggagggccgctcttttcagaggcatcttgcaaatggttaagaacgagccctccttgaggttccttgctaagtaagtttataagctccattttagttgggacagattaagcacaaacttgtttaaagcaataagataatttactggctcactggtcaaccccaggaccaatgggcctatcatggggactgcctctctctgcaccacacccaccctcctgcaagaggtcgacccccccatcctctcccagctgctgacaggtacctgggtatcctcagctcaggctgttcgccccacactatccccacagccaggcctcccagggtacacgtcccgacccccaggggtgtccccagcactgataataggcagagatgtccagagttgcctgagccacttcttggtgttgcagacctcaggctggggcggctcctcctccgtgtggccccggatcagcacaccaggctgctgcctttcgctttttacaggtacctccacccacagggctggtcagggctgggcagtgtttcccagacccccatctcagcacctctgggtcccgccagatgggaagggttgtctgtgcctctgctccacagatgagcagtatcccttggcatcacctgctacctttccagcagtctgtagccatttgtcactatgtctttacctctagtcttctctcctacttccatgaagacgcggccatcagggaagaggccttcctgcatgttgctgtggacatgtacttgaagctggtccagctcttcgtggctggggatacaagcacagtttcacctccagctggcaggagcctggagctcaagggtcaggcaggtgcaagggccagtcccacctccaggggagctccccccagccggaggctccttctgccaaagaatgttccggcacagcatgcagactatgggggacacaccagccctgtttctgtatgtcttctaacctgtgagtttgcctgttttctctctagggcaaccccgtggaactgataacaaaagctcgtctttttctgctgcagttaatacctcggtgcccgaaaaagagcttctcacacgtggcagaggtaacgtcaagatgcccaccttgggccatgtgggggacatgagaattgacagctgcctgggccatgtgcctgcctggctggcaatacaactcgactatttctgccagagcccctcccctgtggtctgaggcctagtgggcggcatgggctgaggacctgctcctctctcacagctgctggctgatcgtggggactgcgacccagaggtgagcgccgccctccagagcagacagcaggctgcccctgacgctgacctgtcccaggagcctcatctcttctgacgggacctgccactgcacaccagcccagctcccgtgtaaataatttattacaagcataacatggagctcttgttgcactaaaaagtggattacaaatctcctcgactgctttagtggggaaaggaatcaattatttatgaactgtccggccccgagtcactcagcgtttgcgggaaaataaaccactggtcccagagcagaggaaggctacttgagccggacaccaagcccgcctccagcaccaagggcgggcagcaccctccgaccctcccatgcgggtgcacacgaagggtgaggctgacacagccactgcggagtccaggctgctagaggtgctcatcctcactgccgtcctcaggtgggttcgggcttcaccgcctggccctctgtggtcacagaggggctcggtggcccaggtggtggttccgcctccaggggcagggccttgtcctgggtctgtgtcagcgggtgcaccatggacatgtgtacattgaggttgtgggccttctcaaaccgccggccacactggtcacaggcaaagtccagctcagtctcagccttgtgtttggtcatgtggtacttgagggatgcccgctgcctgcactggaacccacagacctcacactgcaaaggcttggctcccgaatgtcgcatttggtggacgagaaggtgcttccgctgcttgaaggtttgtccacattcgtcacagatatagttccgcacctctgtgtggatgagcttcacgtggcgctgcaggtagcggtcgatcatgaaaaccttgttgcagccagggtgggggcagggccgctcccggacctcctcgtggtgctccttgatgtgcttcttcatgccgtcagcgcctcggtacacggccgtgcagccctggtaaggacacttgtagatggtgggaagctcctccctctcacaacgaagcttcttcttccatccgggcttgggtcccggcttcttccgaattcttggttcttcagacttcttggcttctttgctttcactcttcttaccagagactttcctttctgggtaaggctcaaaggactcgtccgaagactgggcattttgcttcttgtcattttcatcttcactcaagacgtctccctcagaaaggtcactgaactcgtcttttacccgatcatccgaggttgaagatggaagctgcttctcacccaactgccctggggccctgcaaaggggcaggcttggctgaggtgggaagcccgacctgggccccaccgcgtcgctgtccgaaggaggctgggccacatccgtgctgggcagggtcttggtctcagccccaactggggtccctgtccctctaccctgggaggtctgaggggcatccccagggttccaccctcggtgctggggcagccgtggcgccgtctctttgtcccatggccacttgactgccagcgcactgtccagcaagaaggccttgcagctggagctggtatccatggtgtagtcgtggccctggtcgcagccccacacgacctggatgacgccgcagtactcggaggacagtgtcctctgaaggtggggcagggccccgcagctggccgcatgtccatgcacccaccccaccaagccgtgcaggcactgggggctggatgtgatcagatccaccagacacgctccctcctctgcccctgttgggggctgggcaccgacctttgcacaaggcttccggcgaccagccggggaggcgttgaccctctgcaggaaggacttgagaaggctgtggcactggtagaactgggcgtggcagctcttgcagacaaacggagacaaggtggggtcctggcggacagccacaccaagcaggcgctggaagtcccgtacgagcacgcgctcctctgcggatggcctctccatgctcgctccaggcgccctctcggagatgctgcgcaggcttctcgaggaaaacttcccgtggcagaggcgacagtgacccatggcgagagcccggcctgctccgtgggagacggaggcgcggggcgggcaggcgccggcggaggccacgcggcgcgcaggtggcgggcgggctgcagaaaggggaggggggccggggtctcacgtagagaggggcctggctgccgcggttagacgcccatggcaactccgtgaggggcccttctcgccagccccgtctcaagacggcgaagaggcccggctccgtcgcgacaacccacccggactctgccgcccccgccactaacacccgtggggcccgcagtacgcgcggaggggg

SEQ ID NO: 15236 - RNA, 4095 nt, Homo sapiens
  source 1..4095: mol_type = other RNA
gctgggattacaggcatgagccactgcatccggcctgtgggcctttcttttaatgtcttatttgaggacgtggtgcagcagccttggtgtgggtgctcgaagtccctggcctcctacctgagcctcttctgtccagaggcccagtattaccttctataggtaaaactgtcaccagttttaagacttacaataagcaaagaggaaatgccctcttctgtgctgagggctgtaccctcctacccatgggagcaccaggtcggccattctcagggttggtctcctgcggtttacagagcaccacagacctgccaaaggctttccacgtttgtgcagcaatcctcgagtgtttagagaagaggaagatatcctggctggcactctttcagttgacagagagtggtaagaaacacgctgctgaggcacaaatgcggagggccgctcttttcagaggcatcttgcaaatggttaagaacgagccctccttgaggttccttgctaagtaagtttataagctccattttagttgggacagattaagcacaaacttgtttaaagcaataagataatttactggctcactggtcaaccccaggaccaatgggcctatcatggggactgcctctctctgcaccacacccaccctcctgcaagaggtcgacccccccatcctctcccagctgctgacaggtacctgggtatcctcagctcaggctgttcgccccacactatccccacagccaggcctcccagggtacacgtcccgacccccaggggtgtccccagcactgataataggcagagatgtccagagttgcctgagccacttcttggtgttgcagacctcaggctggggcggctcctcctccgtgtggccccggatcagcacaccaggctgctgcctttcgctttttacaggtacctccacccacagggctggtcagggctgggcagtgtttcccagacccccatctcagcacctctgggtcccgccagatgggaagggttgtctgtgcctctgctccacagatgagcagtatcccttggcatcacctgctacctttccagcagtctgtagccatttgtcactatgtctttacctctagtcttctctcctacttccatgaagacgcggccatcagggaagaggccttcctgcatgttgctgtggacatgtacttgaagctggtccagctcttcgtggctggggatacaagcacagtttcacctccagctggcaggagcctggagctcaagggtcaggcaggtgcaagggccagtcccacctccaggggagctccccccagccggaggctccttctgccaaagaatgttccggcacagcatgcagactatgggggacacaccagccctgtttctgtatgtcttctaacctgtgagtttgcctgttttctctctagggcaaccccgtggaactgataacaaaagctcgtctttttctgctgcagttaatacctcggtgcccgaaaaagagcttctcacacgtggcagaggtaacgtcaagatgcccaccttgggccatgtgggggacatgagaattgacagctgcctgggccatgtgcctgcctggctggcaatacaactcgactatttctgccagagcccctcccctgtggtctgaggcctagtgggcggcatgggctgaggacctgctcctctctcacagctgctggctgatcgtggggactgcgacccagaggtgagcgccgccctccagagcagacagcaggctgcccctgacgctgacctgtcccaggagcctcatctcttctgacgggacctgccactgcacaccagcccagctcccgtgtaaataatttattacaagcataacatggagctcttgttgcactaaaaagtggattacaaatctcctcgactgctttagtggggaaaggaatcaattatttatgaactgtccggccccgagtcactcagcgtttgcgggaaaataaaccactggtcccagagcagaggaaggctacttgagccggacaccaagcccgcctccagcaccaagggcgggcagcaccctccgaccctcccatgcgggtgcacacgaagggtgaggctgacacagccactgcggagtccaggctgctagaggtgctcatcctcactgccgtcctcaggtgggttcgggcttcaccgcctggccctctgtggtcacagaggggctcggtggcccaggtggtggttccgcctccaggggcagggccttgtcctgggtctgtgtcagcgggtgcaccatggacatgtgtacattgaggttgtgggccttctcaaaccgccggccacactggtcacaggcaaagtccagctcagtctcagccttgtgtttggtcatgtggtacttgagggatgcccgctgcctgcactggaacccacagacctcacactgcaaaggcttggctcccgaatgtcgcatttggtggacgagaaggtgcttccgctgcttgaaggtttgtccacattcgtcacagatatagttccgcacctctgtgtggatgagcttcacgtggcgctgcaggtagcggtcgatcatgaaaaccttgttgcagccagggtgggggcagggccgctcccggacctcctcgtggtgctccttgatgtgcttcttcatgccgtcagcgcctcggtacacggccgtgcagccctggtaaggacacttgtagatggtgggaagctcctccctctcacaacgaagcttcttcttccatccgggcttgggtcccggcttcttccgaattcttggttcttcagacttcttggcttctttgctttcactcttcttaccagagactttcctttctgggtaaggctcaaaggactcgtccgaagactgggcattttgcttcttgtcattttcatcttcactcaagacgtctccctcagaaaggtcactgaactcgtcttttacccgatcatccgaggttgaagatggaagctgcttctcacccaactgccctggggccctgcaaaggggcaggcttggctgaggtgggaagcccgacctgggccccaccgcgtcgctgtccgaaggaggctgggccacatccgtgctgggcagggtcttggtctcagccccaactggggtccctgtccctctaccctgggaggtctgaggggcatccccagggttccaccctcggtgctggggcagccgtggcgccgtctctttgtcccatggccacttgactgccagcgcactgtccagcaagaaggccttgcagctggagctggtatccatggtgtagtcgtggccctggtcgcagccccacacgacctggatgacgccgcagtactcggaggacagtgtcctctgaaggtggggcagggccccgcagctggccgcatgtccatgcacccaccccaccaagccgtgcaggcactgggggctggatgtgatcagatccaccagacacgctccctcctctgcccctgttgggggctgggcaccgacctttgcacaaggcttccggcgaccagccggggaggcgttgaccctctgcaggaaggacttgagaaggctgtggcactggtagaactgggcgtggcagctcttgcagacaaacggagacaaggtggggtcctggcggacagccacaccaagcaggcgctggaagtcccgtacgagcacgcgctcctctgcggatggcctctccatgctcgctccaggcgccctctcggagatgctgcgcaggcttctcgaggaaaacttcccgtggcagaggcgacagtgacccatggcgagagcccggcctgctcctgcctcgtccgcgccgtcctcgcccgcgtccccgcaggaccccaccgggccccaggcgcgccgcgccgtcgccccgtccaccctcggcccaccgctaagggaagggcggccccgagtccggctgacgccgccgccgccgtccgaggccccgcactgtcgggacgacccaggagacaggaagcggcccagccggtcccgcttcatggcagcggaggacgccagcagaatcccgcgggtgctgcccggcccgaggttcctagaggacccggcgttaggctccgctcggcgcgctggaagcgaggcggggc

SEQ ID NO: 15237 - RNA, 4029 nt, Homo sapiens
  source 1..4029: mol_type = other RNA
gctgggattacaggcatgagccactgcatccggcctgtgggcctttcttttaatgtcttatttgaggacgtggtgcagcagccttggtgtgggtgctcgaagtccctggcctcctacctgagcctcttctgtccagaggcccagtattaccttctataggtaaaactgtcaccagttttaagacttacaataagcaaagaggaaatgccctcttctgtgctgagggctgtaccctcctacccatgggagcaccaggtcggccattctcagggttggtctcctgcggtttacagagcaccacagacctgccaaaggctttccacgtttgtgcagcaatcctcgagtgtttagagaagaggaagatatcctggctggcactctttcagttgacagagagtggtaagaaacacgctgctgaggcacaaatgcggagggccgctcttttcagaggcatcttgcaaatggttaagaacgagccctccttgaggttccttgctaagtaagtttataagctccattttagttgggacagattaagcacaaacttgtttaaagcaataagataatttactggctcactggtcaaccccaggaccaatgggcctatcatggggactgcctctctctgcaccacacccaccctcctgcaagaggtcgacccccccatcctctcccagctgctgacaggtacctgggtatcctcagctcaggctgttcgccccacactatccccacagccaggcctcccagggtacacgtcccgacccccaggggtgtccccagcactgataataggcagagatgtccagagttgcctgagccacttcttggtgttgcagacctcaggctggggcggctcctcctccgtgtggccccggatcagcacaccaggctgctgcctttcgctttttacaggtacctccacccacagggctggtcagggctgggcagtgtttcccagacccccatctcagcacctctgggtcccgccagatgggaagggttgtctgtgcctctgctccacagatgagcagtatcccttggcatcacctgctacctttccagcagtctgtagccatttgtcactatgtctttacctctagtcttctctcctacttccatgaagacgcggccatcagggaagaggccttcctgcatgttgctgtggacatgtacttgaagctggtccagctcttcgtggctggggatacaagcacagtttcacctccagctggcaggagcctggagctcaagggtcaggcaggtgcaagggccagtcccacctccaggggagctccccccagccggaggctccttctgccaaagaatgttccggcacagcatgcagactatgggggacacaccagccctgtttctgtatgtcttctaacctgtgagtttgcctgttttctctctagggcaaccccgtggaactgataacaaaagctcgtctttttctgctgcagttaatacctcggtgcccgaaaaagagcttctcacacgtggcagaggtaacgtcaagatgcccaccttgggccatgtgggggacatgagaattgacagctgcctgggccatgtgcctgcctggctggcaatacaactcgactatttctgccagagcccctcccctgtggtctgaggcctagtgggcggcatgggctgaggacctgctcctctctcacagctgctggctgatcgtggggactgcgacccagaggtgagcgccgccctccagagcagacagcaggctgcccctgacgctgacctgtcccaggagcctcatctcttctgacgggacctgccactgcacaccagcccagctcccgtgtaaataatttattacaagcataacatggagctcttgttgcactaaaaagtggattacaaatctcctcgactgctttagtggggaaaggaatcaattatttatgaactgtccggccccgagtcactcagcgtttgcgggaaaataaaccactggtcccagagcagaggaaggctacttgagccggacaccaagcccgcctccagcaccaagggcgggcagcaccctccgaccctcccatgcgggtgcacacgaagggtgaggctgacacagccactgcggagtccaggctgctagaggtgctcatcctcactgccgtcctcaggtgggttcgggcttcaccgcctggccctctgtggtcacagaggggctcggtggcccaggtggtggttccgcctccaggggcagggccttgtcctgggtctgtgtcagcgggtgcaccatggacatgtgtacattgaggttgtgggccttctcaaaccgccggccacactggtcacaggcaaagtccagctcagtctcagccttgtgtttggtcatgtggtacttgagggatgcccgctgcctgcactggaacccacagacctcacactgcaaaggcttggctcccgaatgtcgcatttggtggacgagaaggtgcttccgctgcttgaaggtttgtccacattcgtcacagatatagttccgcacctctgtgtggatgagcttcacgtggcgctgcaggtagcggtcgatcatgaaaaccttgttgcagccagggtgggggcagggccgctcccggacctcctcgtggtgctccttgatgtgcttcttcatgccgtcagcgcctcggtacacggccgtgcagccctggtaaggacacttgtagatggtgggaagctcctccctctcacaacgaagcttcttcttccatccgggcttgggtcccggcttcttccgaattcttggttcttcagacttcttggcttctttgctttcactcttcttaccagagactttcctttctgggtaaggctcaaaggactcgtccgaagactgggcattttgcttcttgtcattttcatcttcactcaagacgtctccgatcatccgaggttgaagatggaagctgcttctcacccaactgccctggggccctgcaaaggggcaggcttggctgaggtgggaagcccgacctgggccccaccgcgtcgctgtccgaaggaggctgggccacatccgtgctgggcagggtcttggtctcagccccaactggggtccctgtccctctaccctgggaggtctgaggggcatccccagggttccaccctcggtgctggggcagccgtggcgccgtctctttgtcccatggccacttgactgccagcgcactgtccagcaagaaggccttgcagctggagctggtatccatggtgtagtcgtggccctggtcgcagccccacacgacctggatgacgccgcagtactcggaggacagtgtcctctgaaggtggggcagggccccgcagctggccgcatgtccatgcacccaccccaccaagccgtgcaggcactgggggctggatgtgatcagatccaccagacacgctccctcctctgcccctgttgggggctgggcaccgacctttgcacaaggcttccggcgaccagccggggaggcgttgaccctctgcaggaaggacttgagaaggctgtggcactggtagaactgggcgtggcagctcttgcagacaaacggagacaaggtggggtcctggcggacagccacaccaagcaggcgctggaagtcccgtacgagcacgcgctcctctgcggatggcctctccatgctcgctccaggcgccctctcggagatgctgcgcaggcttctcgaggaaaacttcccgtggcagaggcgacagtgacccatggcgagagcccggcctgctccgtgggagacggaggcgcggggcgggcaggcgccggcggaggccacgcggcgcgcaggtggcgggcgggctgcagaaaggggaggggggccggggtctcacgtagagaggggcctggctgccgcggttagacgcccatggcaactccgtgaggggcccttctcgccagccccgtctcaagacggcgaagaggcccggctccgtcgcgacaacccacccggactctgccgcccccgccactaacacccgtggggcccgcagtacgcgcggaggggg

SEQ ID NO: 15238 - RNA, 4063 nt, Homo sapiens
  source 1..4063: mol_type = other RNA
gctgggattacaggcatgagccactgcatccggcctgtgggcctttcttttaatgtcttatttgaggacgtggtgcagcagccttggtgtgggtgctcgaagtccctggcctcctacctgagcctcttctgtccagaggcccagtattaccttctataggtaaaactgtcaccagttttaagacttacaataagcaaagaggaaatgccctcttctgtgctgagggctgtaccctcctacccatgggagcaccaggtcggccattctcagggttggtctcctgcggtttacagagcaccacagacctgccaaaggctttccacgtttgtgcagcaatcctcgagtgtttagagaagaggaagatatcctggctggcactctttcagttgacagagagtggtaagaaacacgctgctgaggcacaaatgcggagggccgctcttttcagaggcatcttgcaaatggttaagaacgagccctccttgaggttccttgctaagtaagtttataagctccattttagttgggacagattaagcacaaacttgtttaaagcaataagataatttactggctcactggtcaaccccaggaccaatgggcctatcatggggactgcctctctctgcaccacacccaccctcctgcaagaggtcgacccccccatcctctcccagctgctgacaggtacctgggtatcctcagctcaggctgttcgccccacactatccccacagccaggcctcccagggtacacgtcccgacccccaggggtgtccccagcactgataataggcagagatgtccagagttgcctgagccacttcttggtgttgcagacctcaggctggggcggctcctcctccgtgtggccccggatcagcacaccaggctgctgcctttcgctttttacaggtacctccacccacagggctggtcagggctgggcagtgtttcccagacccccatctcagcacctctgggtcccgccagatgggaagggttgtctgtgcctctgctccacagatgagcagtatcccttggcatcacctgctacctttccagcagtctgtagccatttgtcactatgtctttacctctagtcttctctcctacttccatgaagacgcggccatcagggaagaggccttcctgcatgttgctgtggacatgtacttgaagctggtccagctcttcgtggctggggatacaagcacagtttcacctccagctggcaggagcctggagctcaagggtcaggcaggtgcaagggccagtcccacctccaggggagctccccccagccggaggctccttctgccaaagaatgttccggcacagcatgcagactatgggggacacaccagccctgtttctgtatgtcttctaacctgtgagtttgcctgttttctctctagggcaaccccgtggaactgataacaaaagctcgtctttttctgctgcagttaatacctcggtgcccgaaaaagagcttctcacacgtggcagaggtaacgtcaagatgcccaccttgggccatgtgggggacatgagaattgacagctgcctgggccatgtgcctgcctggctggcaatacaactcgactatttctgccagagcccctcccctgtggtctgaggcctagtgggcggcatgggctgaggacctgctcctctctcacagctgctggctgatcgtggggactgcgacccagaggtgagcgccgccctccagagcagacagcaggctgcccctgacgctgacctgtcccaggagcctcatctcttctgacgggacctgccactgcacaccagcccagctcccgtgtaaataatttattacaagcataacatggagctcttgttgcactaaaaagtggattacaaatctcctcgactgctttagtggggaaaggaatcaattatttatgaactgtccggccccgagtcactcagcgtttgcgggaaaataaaccactggtcccagagcagaggaaggctacttgagccggacaccaagcccgcctccagcaccaagggcgggcagcaccctccgaccctcccatgcgggtgcacacgaagggtgaggctgacacagccactgcggagtccaggctgctagaggtgctcatcctcactgccgtcctcaggtgggttcgggcttcaccgcctggccctctgtggtcacagaggggctcggtggcccaggtggtggttccgcctccaggggcagggccttgtcctgggtctgtgtcagcgggtgcaccatggacatgtgtacattgaggttgtgggccttctcaaaccgccggccacactggtcacaggcaaagtccagctcagtctcagccttgtgtttggtcatgtggtacttgagggatgcccgctgcctgcactggaacccacagacctcacactgcaaaggcttggctcccgaatgtcgcatttggtggacgagaaggtgcttccgctgcttgaaggtttgtccacattcgtcacagatatagttccgcacctctgtgtggatgagcttcacgtggcgctgcaggtagcggtcgatcatgaaaaccttgttgcagccagggtgggggcagggccgctcccggacctcctcgtggtgctccttgatgtgcttcttcatgccgtcagcgcctcggtacacggccgtgcagccctggtaaggacacttgtagatggtgggaagctcctccctctcacaacgaagcttcttcttccatccgggcttgggtcccggcttcttccgaattcttggttcttcagacttcttggcttctttgctttcactcttcttaccagagactttcctttctgggtaaggctcaaaggactcgtccgaagactgggcattttgcttcttgtcattttcatcttcactcaagacgtctccgatcatccgaggttgaagatggaagctgcttctcacccaactgccctggggccctgcaaaggggcaggcttggctgaggtgggaagcccgacctgggccccaccgcgtcgctgtccgaaggaggctgggccacatccgtgctgggcagggtcttggtctcagccccaactggggtccctgtccctctaccctgggaggtctgaggggcatccccagggttccaccctcggtgctggggcagccgtggcgccgtctctttgtcccatggccacttgactgccagcgcactgtccagcaagaaggccttgcagctggagctggtatccatggtgtagtcgtggccctggtcgcagccccacacgacctggatgacgccgcagtactcggaggacagtgtcctctgaaggtggggcagggccccgcagctggccgcatgtccatgcacccaccccaccaagccgtgcaggcactgggggctggatgtgatcagatccaccagacacgctccctcctctgcccctgttgggggctgggcaccgacctttgcacaaggcttccggcgaccagccggggaggcgttgaccctctgcaggaaggacttgagaaggctgtggcactggtagaactgggcgtggcagctcttgcagacaaacggagacaaggtggggtcctggcggacagccacaccaagcaggcgctggaagtcccgtacgagcacgcgctcctctgcggatggcctctccatgctcgctccaggcgccctctcggagatgctgcgcaggcttctcgaggaaaacttcccgtggcagaggcgacagtgacccatggcgagagcccggcctgctcctgcctcgtccgcgccgtcctcgcccgcgtccccgcaggaccccaccgggccccaggcgcgccgcgccgtcgccccgtccaccctcggcccaccgctaagggaagggcggccccgagtccggctgacgccgccgccgccgtccgaggccccgcactgtcgggacgacccaggagacaggaagcggcccagccggtcccgcttcatggcagcggaggacgccagcagaatcccgcgggtgctgcccggcccgaggttcctagaggacccggcgttaggctccgctcggcgcgctggaagcgaggcggggc

SEQ ID NO: 15239 - RNA, 3969 nt, Homo sapiens
  source 1..3969: mol_type = other RNA
gctgggattacaggcatgagccactgcatccggcctgtgggcctttcttttaatgtcttatttgaggacgtggtgcagcagccttggtgtgggtgctcgaagtccctggcctcctacctgagcctcttctgtccagaggcccagtattaccttctataggtaaaactgtcaccagttttaagacttacaataagcaaagaggaaatgccctcttctgtgctgagggctgtaccctcctacccatgggagcaccaggtcggccattctcagggttggtctcctgcggtttacagagcaccacagacctgccaaaggctttccacgtttgtgcagcaatcctcgagtgtttagagaagaggaagatatcctggctggcactctttcagttgacagagagtggtaagaaacacgctgctgaggcacaaatgcggagggccgctcttttcagaggcatcttgcaaatggttaagaacgagccctccttgaggttccttgctaagtaagtttataagctccattttagttgggacagattaagcacaaacttgtttaaagcaataagataatttactggctcactggtcaaccccaggaccaatgggcctatcatggggactgcctctctctgcaccacacccaccctcctgcaagaggtcgacccccccatcctctcccagctgctgacaggtacctgggtatcctcagctcaggctgttcgccccacactatccccacagccaggcctcccagggtacacgtcccgacccccaggggtgtccccagcactgataataggcagagatgtccagagttgcctgagccacttcttggtgttgcagacctcaggctggggcggctcctcctccgtgtggccccggatcagcacaccaggctgctgcctttcgctttttacaggtacctccacccacagggctggtcagggctgggcagtgtttcccagacccccatctcagcacctctgggtcccgccagatgggaagggttgtctgtgcctctgctccacagatgagcagtatcccttggcatcacctgctacctttccagcagtctgtagccatttgtcactatgtctttacctctagtcttctctcctacttccatgaagacgcggccatcagggaagaggccttcctgcatgttgctgtggacatgtacttgaagctggtccagctcttcgtggctggggatacaagcacagtttcacctccagctggcaggagcctggagctcaagggtcaggcaggtgcaagggccagtcccacctccaggggagctccccccagccggaggctccttctgccaaagaatgttccggcacagcatgcagactatgggggacacaccagccctgtttctgtatgtcttctaacctgtgagtttgcctgttttctctctagggcaaccccgtggaactgataacaaaagctcgtctttttctgctgcagttaatacctcggtgcccgaaaaagagcttctcacacgtggcagaggtaacgtcaagatgcccaccttgggccatgtgggggacatgagaattgacagctgcctgggccatgtgcctgcctggctggcaatacaactcgactatttctgccagagcccctcccctgtggtctgaggcctagtgggcggcatgggctgaggacctgctcctctctcacagctgctggctgatcgtggggactgcgacccagaggtgagcgccgccctccagagcagacagcaggctgcccctgacgctgacctgtcccaggagcctcatctcttctgacgggacctgccactgcacaccagcccagctcccgtgtaaataatttattacaagcataacatggagctcttgttgcactaaaaagtggattacaaatctcctcgactgctttagtggggaaaggaatcaattatttatgaactgtccggccccgagtcactcagcgtttgcgggaaaataaaccactggtcccagagcagaggaaggctacttgagccggacaccaagcccgcctccagcaccaagggcgggcagcaccctccgaccctcccatgcgggtgcacacgaagggtgaggctgacacagccactgcggagtccaggctgctagaggtgctcatcctcactgccgtcctcaggtgggttcgggcttcaccgcctggccctctgtggtcacagaggggctcggtggcccaggtggtggttccgcctccaggggcagggccttgtcctgggtctgtgtcagcgggtgcaccatggacatgtgtacattgaggttgtgggccttctcaaaccgccggccacactggtcacaggcaaagtccagctcagtctcagccttgtgtttggtcatgtggtacttgagggatgcccgctgcctgcactggaacccacagacctcacactgcaaaggcttggctcccgaatgtcgcatttggtggacgagaaggtgcttccgctgcttgaaggtttgtccacattcgtcacagatatagttccgcacctctgtgtggatgagcttcacgtggcgctgcaggtagcggtcgatcatgaaaaccttgttgcagccagggtgggggcagggccgctcccggacctcctcgtggtgctccttgatgtgcttcttcatgccgtcagcgcctcggtacacggccgtgcagccctggtaaggacacttgtagatggtgggaagctcctccctctcacaacgaagcttcttcttccatccgggcttgggtcccggcttcttccgaattcttggttcttcagacttcttggcttctttgctttcactcttcttaccagagactttcctttctgggtaaggctcaaaggactcgtccgaagactgggcattttgcttcttgtcattttcatcttcactcaagacgtctccgatcatccgaggttgaagatggaagctgcttctcacccaactgccctggggccctgcaaaggggcaggcttggctgaggtgggaagcccgacctgggccccaccgcgtcgctgtccgaaggaggctgggccacatccgtgctgggcagggtcttggtctcagccccaactggggtccctgtccctctaccctgggaggtctgaggggcatccccagggttccaccctcggtgctggggcagccgtggcgccgtctctttgtcccatggccacttgactgccagcgcactgtccagcaagaaggccttgcagctggagctggtatccatggtgtagtcgtggccctggtcgcagccccacacgacctggatgacgccgcagtactcggaggacagtgtcctctgaaggtggggcagggccccgcagctggccgcatgtccatgcacccaccccaccaagccgtgcaggcactgggggctggatgtgatcagatccaccagacacgctccctcctctgcccctgttgggggctgggcaccgacctttgcacaaggcttccggcgaccagccggggaggcgttgaccctctgcaggaaggacttgagaaggctgtggcactggtagaactgggcgtggcagctcttgcagacaaacggagacaaggtggggtcctggcggacagccacaccaagcaggcgctggaagtcccgtacgagcacgcgctcctctgcggatggcctctccatgctcgctccaggcgccctctcggagatgctgcgcaggcttctcgaggaaaacttcccgtggcagaggcgacagtgacccatggcgagagcccggcctgctccttggacagctcagatcctgcggaccttggctttccactccgctcgctgagccggtgcatcacagcctgggctccacctgtagaggagatgtagcaggagggtccgccaggccaccttccaaaatccgagtgacgggcaggtccgtgcgttcgtgcatttttctgggcagagatggtagatttaatccggttgccacaggggacggcatgcagag

SEQ ID NO: 15240 - RNA, 1241 nt, Homo sapiens
  source 1..1241: mol_type = other RNA
gctgggattacaggcatgagccactgcatcgggccaggacaagcatttgataagccataaaaagtaacctcattccagttaggtacagtcttttgcttctaattgcaccaagctccactgtagacagtattagctcctgagtccattttctccaggataacccacctaagagcaaagacaacttggcaacataagatttctgttttccttgtctggagtctcctccttcgaaaccaccttctatatcattcattatagacagctcagaaatacaaacctgactgtatgatttaaaacgccttaatgacttaatacctacaggatgaagtcaaaattatttggcaagagtcacagaatcctccataatctggctcactctaaattcactttgcactaggacaggggcaggcaaaccttttctgaaagggctacatattaattaggctttgcaggccataggtctctatcacaactactcaattctgctcttgcagcatggcagtcgccataaacaacatgtaaacaaatgagcatggctgtgttccaatgagactttattggcagtgggccagatttgggtagtctgctaactctaaactagaattcaacctcatcttaaaatctttcagatgggtgaatggaaactgaccattctctgatgatgaactatttttcttacaacaataaagagtcagagtactcatggtacgtattttaattacaaggtgtcaacatacagattagcataagcttcaactgtcataagaaacatgttccatcaaattcagaaacagcaggtatcagtgaaactggagcaagcattttgaagacttcaacgtattggatggaatttttcaaaaatttcaccatatgttttcttatcttcttcaggaaaatcctctggatgtaatttcatatatccaaacatttcacggtccctcacagcatacaggtagtcagccgtcgcgatcggcctccgccggattaggttatcaatcaggccggagcagtagcccaagaagccgatgtagaggagccgcgggtcggtcagcttgggcgggggcaggctccgggcctcatccggcagaaaccgtaagggttctgggttccgccgtgcgatcatggtgacgccgtttccacttgaggcctggtctcagaccacgaactacaaggaaaaccacgacgaccactaccccggcctaagcggtcagctttctcctcctcctctgcgcgccggactc

SEQ ID NO: 15241 - RNA, 1310 nt, Homo sapiens
  source 1..1310: mol_type = other RNA
gctgggattacaggcatgagccactgcatcgggccaggacaagcatttgataagccataaaaagtaacctcattccagttaggtacagtcttttgcttctaattgcaccaagctccactgtagacagtattagctcctgagtccattttctccaggataacccacctaagagcaaagacaacttggcaacataagatttctgttttccttgtctggagtctcctccttcgaaaccaccttctatatcattcattatagacagctcagaaatacaaacctgactgtatgatttaaaacgccttaatgacttaatacctacaggatgaagtcaaaattatttggcaagagtcacagaatcctccataatctggctcactctaaattcactttgcactaggacaggggcaggcaaaccttttctgaaagggctacatattaattaggctttgcaggccataggtctctatcacaactactcaattctgctcttgcagcatggcagtcgccataaacaacatgtaaacaaatgagcatggctgtgttccaatgagactttattggcagtgggccagatttgggtagtctgctaactctaaactagaattcaacctcatcttaaaatctttcagatgggtgaatggaaactgaccattctctgatgatgaactatttttcttacaacaataaagagtcagagtactcatggtacgtattttaattacaaggtgtcaacatacagattagcataagcttcaactgtcataagaaacatgttccatcaaattcagaaacagcaggtatcagtgaaactggagcaagcattttgaagacttcaacgtattggatggaatttttcaaaaatttcaccatatgttttcttatcttcttcaggaaaatcctctggatgtaatttcatatatccaaacatttcacggtccctcacagcatacaggtagtcttcacgttttacaagataatatccagcaaaaaaaaaggccgtaatatatagaagctggcgatgcaaaccagccgtcgcgatcggcctccgccggattaggttatcaatcaggccggagcagtagcccaagaagccgatgtagaggagccgcgggtcggtcagcttgggcgggggcaggctccgggcctcatccggcagaaaccgtaagggttctgggttccgccgtgcgatcatggtgacgccgtttccacttgaggcctggtctcagaccacgaactacaaggaaaaccacgacgaccactaccccggcctaagcggtcagctttctcctcctcctctgcgcgccggactc

SEQ ID NO: 15242 - RNA, 1103 nt, Homo sapiens
  source 1..1103: mol_type = other RNA
gctgggattacaggcatgagccactgcatcgggccaggacaagcatttgataagccataaaaagtaacctcattccagttaggtacagtcttttgcttctaattgcaccaagctccactgtagacagtattagctcctgagtccattttctccaggataacccacctaagagcaaagacaacttggcaacataagatttctgttttccttgtctggagtctcctccttcgaaaccaccttctatatcattcattatagacagctcagaaatacaaacctgactgtatgatttaaaacgccttaatgacttaatacctacaggatgaagtcaaaattatttggcaagagtcacagaatcctccataatctggctcactctaaattcactttgcactaggacaggggcaggcaaaccttttctgaaagggctacatattaattaggctttgcaggccataggtctctatcacaactactcaattctgctcttgcagcatggcagtcgccataaacaacatgtaaacaaatgagcatggctgtgttccaatgagactttattggcagtgggccagatttgggtagtctgctaactctaaactagaattcaacctcatcttaaaatctttcagatgggtgaatggaaactgaccattctctgatgatgaactatttttcttacaacaataaagagtcagagtactcatggtacgtattttaattacaaggtgtcaacatacagattagcataagcttcaagttttacaagataatatccagcaaaaaaaaaggccgtaatatatagaagctggcgatgcaaaccagccgtcgcgatcggcctccgccggattaggttatcaatcaggccggagcagtagcccaagaagccgatgtagaggagccgcgggtcggtcagcttgggcgggggcaggctccgggcctcatccggcagaaaccgtaagggttctgggttccgccgtgcgatcatggtgacgccgtttccacttgaggcctggtctcagaccacgaactacaaggaaaaccacgacgaccactaccccggcctaagcggtcagctttctcctcctcctctgcgcgccggactc

SEQ ID NO: 15243 - RNA, 2934 nt, Homo sapiens
  source 1..2934: mol_type = other RNA
gctgggattacaggcatgagccactgcatcttttaccttagaaggactatcttgacaggccttggaccactggacccctggaagttttactgagctagaaggtctctaaattttagtcagacttattttccatcctctggcatgcaaacgtctcatgaataagtctggtgtgtttgctatttcttgcttactggattcaatcagcataatgtcatcaatgtaatggaccacagaagtctctgtccatgtgtgagggtgacactcaacttttggcaggatgagcatacaagagtcacaatctcacctgtgtgctgggtgcagttatatgtcaaaatcccacctgagtcacagtatcaatgatgaactggatccatgcatgagagtcccaattccacctgtagactgtgtgttgtgttggccctatgatatgtcacaatccacctccatttgcataacctagagaaaatagaagagtcgcagagccttctgtgactcgtattagagtcaaagccttctagttgtgttgaatcctggtcttagagtcaccatccacctggaatatgtctcaatctcccctgtgggcaaggcccaggctggagaatcagatcacttgcatgcagggcccagtgacatattatattttctctaggcacagcccaggcaggagagtcacaacatttgggtgttgggctcagagatatgtcataatccctttttgggtcatgtctcctaggtgagaagatcagagatgttgccgattctgtgtaagtctcaggaataagagaagagtcaggtatcctagaaactcggctacattatatgttgcaattacccaagtgggcaggaatctcatgagaagagggtcacatcatgtagctgctgagctaaacgatgcatcacaattcccactgtgtattggtcccagaaagaagaggagagtctcatcatctaggtgatgggcctggaaatctggcatatgcatcctaggtgctggatccagtgatatgtcacaatcctcttctttggcatggcacaggaagaagtagagagtcacaccacctaggtgttggaccaagccatatgtcacaatacacaataaatgcagggcctaggtgcttggtccagtaatatgtcaaaattcccttgagaggtgagcccaggcaagagagtcacatcatttcggtgagaaccccacagatgtgtcactattttccctgtgaatagcgctgtgtgctgggcccagtgataagtcactttcccttgtgtgggcatggcttcagcaggagagaagagtcacatcaccaaggttctggttccagagatatgtcacaatctctccttgatgttggacccagccatatatcacaatgcacagcatatccagggctcaagcagggaagaaaaatcacatcgtctagttgctgggtttgatgatatgtcacaatcacttgtttttgcagaacccagacagaaaagaagagtcacatctcctagttcatggatgcagagataagccaaaaggctccttgtgggcaggacccaggcacaaggctctcatgccctaggtgtttgtctcagccatacgtcacattaccaaatatatgcagggcccaggcaaacaaggtgagtcataacaccttggtactaagtttaatgatatgttacaatccccacttttggcagggccaggacgcacacacacacacacacacaaacaaaggcacatcacataggtgattaaaaaaaaaagatatgtcataatatccctgtaagcagggctcatgcataagagtctcatcacctaggttttagacccagagatttgtcacaatacacaatttatgcaagactcagacacaagaggaaagtcacgtaacctaggtgctgggtccagtgatacattagaatctctccttgggtagagtccaagcagtagaaaagagttacattacctgggtacttgctccaggaatatgtcacaatacctcctgtgtgtgaggtccagtgataagccactcttccttttgtgcacacggtccaaacaaaagatgaaagtcacatcacctaggtgctgggcttccagaattgtctcaatccctcagacaattgttgtcttgattcgatcctcttcaagaggtgatttatggtccgctatggaactttgccaggtatttttaaatgcaggtttctgataactttggagactgtcggtaggaagtgagcagcagattcacatcatgtaggttttcggcaaagatatgtcacaatctttcctgaggtcagaaaccacgcagaagtcatctcacctaggtgctcagccacagatatattacaatcccctcttaaagcagagtacaggcagcagagtcatttcacctgggtgctgagcccagtgatatgtcaaaatgctctctgtgggcacagccttggcaggagagacacatcatctggtgactgggtccagcaatacattacaacattttctgcgacatgggacatgtaacctgtgagtaggtagtgagcaggagagtcacatcaactgggtgcttggccagagatttgtacaatattccctgatggaagggaccaggcaggagaggaacatcacctgggtgctgagcccagtggcatgtcacaatgctccctcaactaggttctgggtccagtgaattgctacaatctccttttttctttggcagtgcccaggcagaagagaagaggcaaataacaatctcaactgtggacttgatctgtgtatgagaccttccatccatcctctagactgtgtctccttagtggactcacggtttctcaagtctcaggggtgctgaatcttggtctgagagttaccagcttacttgtacactggattcaaggatgaaagtcaatttttcaacttttgaaactttcattggttttgagattcagaatctc

SEQ ID NO: 15244 - RNA, 4036 nt, Homo sapiens
  source 1..4036: mol_type = other RNA
gctgggattacaggcatgagccactgcatgcagccatcttttttgataaattatagttatttagtccttgaatacagacgttctgtcacatagtgcttgctatccacttttggatcatatatgttattcagtgttttcccctcttagtgagaagactatcttaagttgacttttcattcaatctccaaggatctgaaaagatggttctgtgatcataattaagaaagcatcaggaaatgggtcaaatatcagcagggatgaccaataaggtaaattacttactttgactctttttcactcaggtctacatcatcataaataataacttcctgagacttaagttctagggtcaagacagaatcaaaatagtccattattaagcatggtttatataagcactgactttccaaattatactcaattacctaattatccaggtgcatcttcaggtctgttttagcaaaatctgatcataaaatacagataggctagaagaatcaaagaataaaaatattctctatttgggaagaaattcaactgaaagattaaaaaaaagtgtgatgtcccagtatctcaaaacatatatatttatattaatttgcttttacatagagttccagaaaaatatgagttgctcaaagagtcatttttagactaagttcccatctttctggaattgaacaaatatgctatactgctagaatagtgagaggtcttttcttaactcctaggggggagaaacagcttaatagaacagtaatgttgatttttcttccatggtttttatttcaaatcattggcaattgctcctatacaataatcttgcataatgttgaatctgactcagtgcataataataattaggcattttcattttaggatattcacattccttggcactctacatagaattacatgattttcatttgattcaccactgaacaagtttgagaccttctagtataattattcataattattcactcccttattttattaaataccttcaaatgtgggtggggatacaatgcatgcctattctaggtcagcttttttcttttaaacacagaccaaggatatgttgagatgtgggattttatcaggtatatataattgtcatttgtcttttagttcagcaaactcatatttatgaaatataatatacttttgaattgtcaagttcgagtgacatccaggtagccacatagctagaacccctaaacaaaaactaacaaacaacagaacacatgaccctcttttattgacaaattcaatgtactgaacgtgtattgacagcctactatgtgtcaagcaccgtgctaatttatgcactattattttaatggaaaagcaaacaacattccaatgatccattctcaattcagttagtttgctggtggcaatgtgatcatattcagttagtgtcttaattaggatgaaggatatcaagtccttcaaaaggcagtatggtagaatgcaaaatgcatgagtttcatagtcagagagcctggaatacaaatcctggatcacttaaatatggtcctacagcttctctaaaaagggatgataacatttatttttctgggattttaagaggaacacatctgccccagggcatggtatgtagtaggtacttgagaaacactactcatcttctccaaagtaaaaaaatacttccgtgtgaaacatcttctttgattttggtagagcaatttttcatcaaatgtgggaatgcaggaagggttaccatttctctttccctgcctctgaatatacaaaagctgagtacttttggtctgcaataagcaaatggcacttacctaaatcaggcagcaaaatggaaaatgcacttaagttttctttcgacttggttttctttattttaaatctatccttttctttcttgaagaattgctgcagtcttttgagtgcttcttttccatctaaatctatctttgggtagttgttctttgttttgtagacatcttcatacagttctctattttcttcactacttgaggcaagtgagctagagtagttcagcttcggtacctctttcctggagtactcgacatcatcatatatctcctccgagatggaacttgtcttagagacccctaggtctggagtttctttagttgactccaaaacctccagatgcccacagtggccttgggagtgcctggccagctttgggccctcagggcagggatttgtctggatgatgtcaatcatggcctcttgctttccagccaacatgttccttctacctgtgtggacgttggtcatctgaattttttcaggtgtcccttcacaggcatctaccttgaaaacatggtttgaatatggttccttttctgtgtttttaggtttcaattcacatggttgtttttccttcatttttttatcttcatgtttagcactaggttctggatagggaaaattcttcccaggcttttggagttcttcaattccaacttcataagttgagttctggaggctggaagttccaagatcaaagtgacaacagattcctggttcatagacagctgtcttctcactgtgccgatcagcaatttcttttgcagtgcacaggttaatggagttgccagagtgtctcagatatgaaattgttgcctcgtaattatgtggttcttcaaattctgcattgaaaagcctctctggagacagggagccctcttccacagtcacttccccctgagtcttgggaacagcagctggctgcctctgaaaggcctggaggttcacgatgggaggtcttgaaggctttgggggaggaggacccagggagtcgatggagggcaatggctttgttttgggaaggtggtgatgcctgacatctggctgtttttctggggcctgactggcaagctcacactcatagatgggctggcaggggctgcttgccgggctcctctcaggaggtgggttttcccagctttttctgatatgttgagaaattacaaaagagggatcttcagagacgttatgtaatattttgggggccaccacgtgcttctgggaaggaagagtctgggctccttttgtttccagctttttcctgggttcctctggagtaagccccatgcctttttgcccttccagatggatggccttacttccatagttggcaaggagaagggctgaagacatttcacttttctgagatgaaaccttctcccagttccagagtttgtttctgaagctattggccaccattactttttccttagtgattatctcaacatttgattgagtcacctctaacagcagagaagccttctgtgaacttgttgcagaacatacagtagactttcccagaggccctggggagttagaacattttggaatttcactcttctgagccaactttattttctgaggttgaagaggctgggactcactactggaacagtatggtgtgcgctgcttgtggttggatgagaggggtttcccattggccaaaatttgagttgactgtgtgcctccaatgtcaccctttggagaaacacctgctgggaatttaataggtcctggaagaggtggagcatcaagattttgaaatttggctcgaagttccttgaagtttcttaccccttccccttccattgctttcctccaaggcagagtcagggaaacaagcccagcctctcagagctgggtcctggggccaacaatccgctttcctctgtctctgctagccagggagcaatcacttcccacaggacacacctgagcccaggctccccacctgccccatctgggccgaggctcctcccttgcctggggctgggccagggccggccgccatcctcccagcttggcttagaccagcacctgcaggggactggggagagtactccacctgcagtcctgccaagcccacctcttctcagcaagcggctcttcccgttgctcccctccggctggtctgacagtcactcactctccagggcatttgtgcccaggcagcaggagctgtgaaggaatggggatggcaggctcctgttagtac

SEQ ID NO: 15245 - RNA, 2441 nt, Homo sapiens
  source 1..2441: mol_type = other RNA
gctgggattacaggcatgagccactgcatgcagccatcttttttgataaattatagttatttagtccttgaatacagacgttctgtcacatagtgcttgctatccttcatgttgtcatgtacattggagataatttaaaaaatgtgttgaaatgagtttcaagttttgactctttttcactcaggtctacatcatcataaataataacttcctgagacttaagttctaaatcaggcagcaaaatggaaaatgcacttaagttttctttcgacttggttttctttattttaaatctatccttttctttcttgaagaattgctgcagtcttttgagtgcttcttttccatctaaatctatctttgggtagttgttctttgttttgtagacatcttcatacagttctctattttcttcactacttgaggcaagtgagctagagtagttcagcttcggtacctctttcctggagtactcgacatcatcatatatctcctccgagatggaacttgtcttagagacccctaggtctggagtttctttagttgactccaaaacctccagatgcccacagtggccttgggagtgcctggccagctttgggccctcagggcagggatttgtctggatgatgtcaatcatggcctcttgctttccagccaacatgttccttctacctgtgtggacgttggtcatctgaattttttcaggtgtcccttcacaggcatctaccttgaaaacatggtttgaatatggttccttttctgtgtttttaggtttcaattcacatggttgtttttccttcatttttttatcttcatgtttagcactaggttctggatagggaaaattcttcccaggcttttggagttcttcaattccaacttcataagttgagttctggaggctggaagttccaagatcaaagtgacaacagattcctggttcatagacagctgtcttctcactgtgccgatcagcaatttcttttgcagtgcacaggttaatggagttgccagagtgtctcagatatgaaattgttgcctcgtaattatgtggttcttcaaattctgcattgaaaagcctctctggagacagggagccctcttccacagtcacttccccctgagtcttgggaacagcagctggctgcctctgaaaggcctggaggttcacgatgggaggtcttgaaggctttgggggaggaggacccagggagtcgatggagggcaatggctttgttttgggaaggtggtgatgcctgacatctggctgtttttctggggcctgactggcaagctcacactcatagatgggctggcaggggctgcttgccgggctcctctcaggaggtgggttttcccagctttttctgatatgttgagaaattacaaaagagggatcttcagagacgttatgtaatattttgggggccaccacgtgcttctgggaaggaagagtctgggctccttttgtttccagctttttcctgggttcctctggagtaagccccatgcctttttgcccttccagatggatggccttacttccatagttggcaaggagaagggctgaagacatttcacttttctgagatgaaaccttctcccagttccagagtttgtttctgaagctattggccaccattactttttccttagtgattatctcaacatttgattgagtcacctctaacagcagagaagccttctgtgaacttgttgcagaacatacagtagactttcccagaggccctggggagttagaacattttggaatttcactcttctgagccaactttattttctgaggttgaagaggctgggactcactactggaacagtatggtgtgcgctgcttgtggttggatgagaggggtttcccattggccaaaatttgagttgactgtgtgcctccaatgtcaccctttggagaaacacctgctgggaatttaataggtcctggaagaggtggagcatcaagattttgaaatttggctcgaagttccttgaagtttcttaccccttccccttccattgctttcctccaaggcagagtcagggaaacaagcccagcctctcagagctgggtcctggggccaacaatccgctttcctctgtctctgctagccagggagcaatcacttcccacaggacacacctgagcccaggctccccacctgccccatctgggccgaggctcctcccttgcctggggctgggccagggccggccgccatcctcccagcttggcttagaccagcacctgcaggggactggggagagtactccacctgcagtcctgccaagcccacctcttctcagcaagcggctcttcccgttgctcccctccggctggtctgacagtcactcactctccagggcatttgtgcccaggcagcaggagctgtgaaggaatggggatggcaggctcctgttagtac

SEQ ID NO: 15246 - RNA, 255 nt, Homo sapiens
  source 1..255: mol_type = other RNA
gctgggattacaggcatgagccactgcatgcagctgacacataattatgtctgttgaatttaacaaaacatttggtttgtattttaaaattttttgtaattcacttcattcattcactcattcatttaagacagaatctcgttctgttgcccaggctggagtgcagtggtgtgatcttggctcactgcaatctccgtgtcctgggttcaaatgattctcgtgcctcagccgaatagctgggattacaggtgtgca

SEQ ID NO: 15247 - RNA, 508 nt, Homo sapiens
  source 1..508: mol_type = other RNA
gctgggattacaggcatgagccactgcatgcggccaggaagatatttcttaattgtaattaagatgtagatgcatgcatgtccaccctttctgtataagtgatactggagcatgtatcaagatggaggaccactggaaactcattttggacacagtaacttaaatgaggactccttattacagcagcatgtattagtatatcagttacatttggtataatgtcattgttagcgcaggaacgggaggaaaaacggacggaggcggctctacagcaacacaggtttaccgaacaaacacccgcggagggggacaccaactaaggccagagcccgcccccgcttacagactgggtaagtttaggtccgggtgggagagatctgggcttgttgtgaagtggggtgggcagggtggttagctgttgctaagtgaggaatttcctgagatcaggcggttgggcttaggacttgcccggcaggatgtttctcacagcctgagccctaggggaatt

SEQ ID NO: 15248 - RNA, 2705 nt, Homo sapiens
  source 1..2705: mol_type = other RNA
gctgggattacaggcatgagccactgcgccaggacaaagcataactttaaaaagcaaaaatgtattaacagcactacatatttacttctctgcatttagaggagatacatagatggctggctgatagaggggaagtggttagctttgttaaactttagccaaagttattaatgctgcttttcatgaatcactgtagcaatgcctttcttcttgatatttaggaaagtagtctggtttttggagtctctacctgatgactgcctactaatctattagatcattaaggactattttgagatacaagatcatacaaatcataagctttgcttccaatcactctcacttgtagggccagagaaatggactactcaggagctacagagctctctgattggctgaagacccagagaaactgtggattatgcaagaactaacaaacatatggagactaagttcccaaagaagagttaaatatctttgagtttaaaccctatctacagctgtgtttgctggaattgtcaggactgtaatagagtttcagttaccaaggagaaatgttgatttagagaaggggtcagccaactttttctgtaaagggccagctagtaaatattttggacttaaccagccatatggtcttctataatcattcaactctgccattgtagcacaaaagcggccatggacaatatgtaaacaagtgaatgttgctctattccaataaaactttatttacaaaataagacagcaagccagatttgacgcgtgggttgtaatttatcaatctattctctatagtgatggctgtcacactctatatgtacatcagaatcacctatggaactagtttaaaaggtaggttcctaggctccagcctacccctacagaatcagaatctctaggaatgcgaatcagcaattcaataaggtccacaagtggtgtgtgaaccacacttttaaagctttgtgttatgcagctagcttcatctaagctggggtggccttgctgtcctagatgtgggccagcacttcctgcatcctgtggcagtaaaaatggagtaacttttattttctttgaccttcctagtagaaacaactgtttttgtttgtttgtttgttttttgcttccaacctctaaaatgcataaaatagtccttctcaggtgaaattaacatgaagtttagggatgattttgaatgaaaatgctcaacttaaaataacaagattttaggccgggcgtggtggctcacgcctgtaatcccagcactttgggaggccaaggcgggcgaatcacgaggtcaggagatccagaccatcctggctaacacggcgaaacctcatctctactaaaaatacaaaaaattagccgggcgtgatggcgggctcctgtagtcccagctactcaggaggctgaggcaggagaatggagtgaaaccgggaggtggagcttgcagtgagctgagatcgcaccactgcactccagcctgggtgacagagtgagactacgtctaaaaaaaaaaaaacaagatttttcaaccaaaaagcttcctgaaatcctttaaattgcaaaattagtaggcacaattcttaccaaaagacagggctacatctgaagaaatagtttccattgttctccctttctctcaaaatacctccagcaaaggcctgccctgttgcttataattccactactaacaagtcattactttgtgtctaggggtctttgcttcaacagaacctcattaaaactcatgtgaaaacagaaagtagaaaatctctgtggtttgcattaagttgacaaaacaaaacaaaacaaaaaccaactctgcaggcctctggcagctgctcccaactttaacaatcagtaaaaaataacttattcagctaagttcagttctgataaaatgaaaaaagtgcttttttatttgtttgtttgaattcccaggaatcaatcacccaatcagtcaacaaggaagtgatgttcagtctcgtgaatagctccaactcttcagctctccagattttcccaacctccctggccctggatgaactcccggatggcttggttcccattgatcatacccgtcatggggatagccacctgtcccactacttcaggagcaatgtgagccatgtactcaagaagtttcactgacactgccagaaaagctctctcataagctaagctggaatcctgagcacaccaggtcttgctgagagattccacagtgtcctggagtatagctcctgtctgtcccttaatggtttctgcaatgacgtttttggcagaagcttccaattctccgttgaactggtcacccaacatccgaaggcgaccagcaatgatagccacatcaaaagaacaaggctctcctgaatctacttcatctacacagcataggttccggctggcaacctgcaatgttgggctcaagaagtccatgagtagagtgttcacaatgcattccgtttgttcctcaaaagtttgggagctcttcattttagatgtttgctgtcaagttttgcttttccacgaaacaagcagttttcagcccagcaggaagttaaaaacactggtaaatcaacaaatgtttctacctcttgtagtttcctgacatgtaatcctggaacttttcccactagctttcttcaaacacagctgctcagaaaggtgggacttctcagaaggattacctacttggaact

SEQ ID NO: 15249 - RNA, 4136 nt, Homo sapiens
  source 1..4136: mol_type = other RNA
gctgggattacaggcatgagccactgcgccaggccgaaataccagatcttcatggcagttgtcttagaggtagagaagaaaacagccagactgagccgggtgtggtggctcatgcctgtaatcccagcactttgggaggctgaggccggcagatcagttgaggttgggagtttgagaccagcctggccaacgtagtgaaaccccgtctccactaaaaatacaaaaattagccaggcatggtggcgggcacctataatcccagctacatgggaggctgaggcaggagaatcgcttgaacctggaaggtggaggttgcagtgagctgagattgcgccactgcactccagcctgggtgacagattgagactccatctcaaaaacaaacaaacaaacaaaaaaaaccagcctgactgaattcagtcacagtaattatacatgagtggttgctagttcctttaaccacaccagaagcattttaaagggaagatgtttcctaactccagtgattttcatgggctgaattccaggcagttcagcaaactcaacaattccggtggtatgagaaagggcattttggagtaggagatttcggctctgcctaggaagatacctcagaaaattcccctcgtgcaatttcactttgcatatgcttctcctgttcttccatttctaatccataaaatcccaaaatgcttgggagggtttattttgattttttttaacaatactgccctgctggcaacagccacgatagtcacttgctcatctgaaaatgccttgcactttctttttcactagcttcgtgtatgacgcaaaacagaaatatttcaattacaggtgactaagagtaagaaaaatatacaactatatttaaaatacttaaattaacaagatagtacttttccattctaacaaaatatcatacattcagtttaaacaagagttaatatccagacacacgttttcaaaatacctgatgctagttgaaaattagtgaccatgaggctttccaagatatttctaattagcaaactgtgtacaattttgaagaagtgtacacaccgtgctggaagacagacactgaacaggtcaaaatgcaaactcatgtatctttcatcaacctaaatcttgttgcttcacttttctaaatgatactttggctgtcagcgaatcttatagcttcttttcccttaaagacaataatatataacaacaccaccccacacaaataaccataaacttctttgtgtgaaataagccctatcaaaatgtgttcatgtatttctgtaccaactgatctatactgagactgtcatgaaaaaggtatcaaacaagtgtaacaggcctacacttaaacctctgcctcaaaggagaaatcagatacttgccacgttattgcaaagtcaaagctgctacacttaaaatatggtagatagtttagaaaaatcaaatcaaaaatgttttctcactggctttttcagataaagaagttggaccacaaaccaacacatctgtgtgaaaacagccaccaatttgagtccccccagcccctcaaaaaggaacaatgccaccagtccctcacaatgaccataacgtctctggccaggactgcgatttctagcgcgtgtcttcacattctatctctggggaagcaagacaaacaggctctacccatttccctccttttgtctccacaagccagcacctaagatcctctgaatttgttcccatccaatcctgcaaacttccaagaagggcagtagataacttttcaaaagaaaaagaaattgcataaggtccctacataatactgaggctgaaacgagaagaggctgtccactgtaaaagcaaggcacttggggcaggagccaggcaggtggcctgagcagggtccctctcagtgagtcaacagtttgaggcgcgtaaaccagctgaccaggagggacggttctgtggacgaggacttcgtagctgaggagccagatttctttttggtcccttcctcctggaatggaatcgtggcgctgctgtggagatctgagttgatgtagcacctgcttcctcggatgtagtccgcaccccggaccagatgccgctcggtcgtgggtctggagaaccggtatgggggagaggagctctcttcaatgatcggaggaatccgctcgttactgaaataccggcaaagggcatcctcccctttcctgccatgacctcgaggtctggcaaaagggtccacaatccccatccagttcccatcagcaggcatggacaaaggccgtggcttgccataagatggtgttttctctctcatttttgtgggcagaatgttggtttccaccgagtacccaggcaactgatccgagtctgcaatggtgaatcttcgtctccggctttcctggtccaagaaggaattcggggactctgaacccttaggaccaggcaatggttgtttgcacttactggaccctccataaacaaaactgccattctcatcccggggagagtagggaacagcaggcggaggaggaatataaagatccaggatggctgacttctccttcttcagtgaggtatccatagtgctttcaggggactgggttgtcgcgggtggaggtgaggtctgtacaagaggtggcttccaccgtaggtttttcaggggagcaggagtaaagttgaaagacccggtggggcgcttcttaagcagtaacacaactccggtgggattctctctcaatttcttcaccagatttttcagctgccatcccaccacagtttgctgattaacttgaatgacttcgtcaccagcatgaatcttctgagatctgtctgcaggagaattttctgtggttccagtaatcacgtgtaacccatcataggttgatttgatgtacatgcccaggccttccccaggtttaatgtttggtaagtgaacttcctccagacatgcacactggctcatcacaggatctgtggtagatcggattgttttgtcacagatgccatttaaaaccttgaccacagttaaaactttatcctccatttccgctacaaagcaatccttctggactgtagtggtcaggtccaagcaaagctggataattttgttcttcgtgactgagaaatcagtgatccctgtaaacggagcccggtccagccacgccagcagggccttggcggcgccgatgagctccaccaccgaggtcaggaactcattgggggccttgcgggaggtgttgccatcgtaagcgggacttttccgtcggctacttatgtaattctgtaaattgtgggaagatgctctcagtttcagaaccaagttcttcatgttatcagtttcgaggccataattcagtgcacagagaaggtccacagcctccaacacaagctcctggtgtccaatccgtgtgacccccagctcctccaggtcctgatgggaaatctgcagcagctgctcgccgttgatcttctctcgttcaaacttgtggacatattgttgcaggcagtcatccaaccctctagtccagtccaccacttgtttggggctccacttggtcacgggttccatggtaaaccgcttcgcctctcgctgggctggagagtcgcagataaagtgctgctgcctgcgctccggtgccccttcccgggagggcgcgcccgcggctgctcccctgcgcccgagcgactccgtcaagactgcatggccgcggtcagccagtcgtcccagcgcggctccgccaggggagcccggccctctccctccagctgccacagtccagctgcagctcctccttcccccgccgccgccgggatcccgggcacagctgctgctcccgagcgacggcagctgcaggcacgccgggctgcgaccccagacccctggcctcggctcggcacgggagcctcccggcccgcgaccacttcctcggatctctcgaggcgcgatcggctctccctcggccggtcttctcgcctgctggctctccggggtccccgctccgcgtgcgctggcgtcccggagccttcccggcgcaggtcccacctcctgcgccgccctcccgtgccgccctggcagggccgagcgcagagcgtgcgcgctcgggttgcaaagtttcagctccggttgctgcaaaccgaat

SEQ ID NO: 15250 - RNA, 4122 nt, Homo sapiens
  source 1..4122: mol_type = other RNA
gctgggattacaggcatgagccactgcgccaggcctcctctttctttaactcttacatgcactccagcctgggtgacagagcaagacatcatctcaaaaaaaaaaaaaaaaaaaagtagggtagtaagttccaggtgtgggggaaccaatgtcagattgttctctgttaatggctgattaccccaagttattttattccataaatcatgacacttgggtttattagtctacccctcccatttttttacagtgcttgaggaaacaaaagatcagaatgtatattgaagaagagaccctaatttatgatttctgagttgagtttgtacatgttaacgtttggtaaaagtctcctgattgaggagaggctgcaactaggccctgattcggagatgaatttatagacagaaaggaaattgtgatggtgatgtgattattgacacatgcacccacccccaaacaggtaatgaccgagaacctgttcctaagatgcgtgtaaaccacatcttcccaggctaagggctccttcatttagcagctcagcatcagggccagtgaagaccgaacctagtgatgtctgagtccacaatcaacttgtatttaggagtggattctactttttccaggtgcaccaaaaacaagcctggcacagtgacagagaaagagtgttctagagagagaaaagtgcaattaggagctaattacattgataaaaattggaatagcgcttacctaaatgattgtccagtttggaaacgctatctgtctccaagcacaaaaactgattcctttactttgcggtgaggagaacatggttttggtattattctgtaaacagtaactgaagaatacaacagtcattgcaagggtgccagtggagagggaggggggccttgcagttgctatcagtttataggcaaggattgaaaagtcacatacaaaagcaacagagagcctcccacaggaggctgagtcattggagttgtgggtgggtgggaggggagtgggcttggaaaccatttaggccaagcccctcagagtggaagggtgttgcccaaggattcgtggtgaatgagtggctgaattgggaccagaactggcttctcttacccttctcctccaccctgctgtgagacaaatggaagaatccagcaacaaaatacctgtcatgggctaaactctgtcttccctaaattcatttgtagaatgaccctcagtacctcagaacatgactgtatttggagatagagcctttaaagaggttatttcatgaaaattaaccaccaattaatcggggatggacccgaatccaatctgactggtgtccttggacaccaggagagggaatgtggacacactgagggacaccagggacacgggcacacagaccacatgaggacacagcgggaaggtagccgtctgcaagccaaggacagaggcctcagaagaaaccaatcctgccaacaccgtgatcttggactccggtacccagaactgtaggaaaattcatgtgcgttatttaagccactcagtctgtggtagttcattgcggcagcccggctgcctgacacaccgcctctccaaggctgcgcacaccagacgtgcagctttctggactacgtgctggagcccacgtgtcgccaccatggctttctgttctcagaacctagcggcgtcttaaagagggcaaggagagagcgggcacagcagcgacacacagcattgctttgctactcaaaatctcaaaaccaaaaacatctaagctaagctgacacttggagagctgaaggggggcatggcttgcagtggcttctgtggacttacggagggtaattgaaaccctcctggctccggtttcccaccagaagaatgggtgtcacactgcctggtcttctggaaaaatctgatttgcccacatctgtcctacacccaggaagcagacactcctctatattaggattaaattggcaaccccccaatgttcacaggcagccttcggagagcagctggattattccaagtctgcctttgtttgcactcaagctgcaccaggtgtcctcaaatccagctcccactcccaggcagcctcttcgaaggcaaccttccacttaggtggtttagacagatgtctacaagattccatcttagggccttggtccggaaatattacccttgtaaggggacagtatccccaggaccagaaacagtgtctggtaataggaactcagaccagcccgattctaaaattctcattgtcagaatcagttatttgggttaaggcataaaaggctcctgtaaaatatgttatcaaagggccatacatattaggatgtcttcagccattaacacctctttgtgacttcatcagtgtggcctcagagccacccttagtcccttagtgccagggcccagggcagctgagttctggtgtgaggaaaggagaaaaagttcaccacagcctgtgtcagggagggaagagcatggacaggtgtgtcatgtggagggacaggggtgacaaggagaaaggagttcagaaggaacactgacagcttgacatgtctaagtcagccagacctctatatcagagtcacctttcggccagatggtgcagatcttgaatgtgaatggccaggccagttggcaagtgcacgagtccagctgcatctgtgtaaggagcttggcatctcagagctggccctggcccagggccatgaagttggggggtgcaggaagaatatacaaagggaacatcggtgtctcctgggcttggggggagctgctggcttcctggagccactgctgtgattggcactcacatgggcggggcttctcccatgttcccagacaatcagcttgcccacagactccagactcccacacccatgctggggcagttagagcccttctggagaagcagggagaggactggggtcaagtgacaacagctaagcatgggtggcctgggcctgtcaaccacaggcctggggctcaggggtcacctggagagaacaggaagggttgtctggccacccacagtccagggatgggggcggccgaggctcagcagggtgaagaggacatctgatcatagtcggggcacttgagcaaggcggggtagttgctgttcatctgcagggaggcctcgctggagatgtcggaggggctgcggcccctgacccaggcgtctgggtgtaggaactggcctgagtaatcggagcagttgctcagccgagggcggtagaagccagggtggggcctgtacatgtcctccgcggtgtaccgcttcataaacaggtacacagacatcaccccggcactctccgttaaaaggaaggagatggcggcgaaggcaaacgaccacccatacttgtagttgaagtaggtctctgcatccttggtcctgttgagcatctcatcgttgatgctggagatgtagagcaccaggcccaccacgagagagaggcctgagaggataaagaagatgccagagacaaaggccagtatcgtccggtggggacggatgtgtccgatgttgttcaggataaacccaatgaacatgaagaagaggctgaccagagggaatggtgtggctgagcggatcatctttagaacattgaccgtggactcggatgtcagctgggtgttcatgggcatcacatattctatggtgaagcaacgcccccgctcctcacctgcaaggaagcagacccgccagaggcctgagtgcagggacatcttgatctcggtgctctggttctggggcacaatcacaccctcctccaggtacagccagtagtcggtgctgaccgcgatacccaggaggcccaagccacagacagcaaagacactgctcagcagggtcagggccttcctcccgcaggcactcatcttcctggaccgttgctgtgcaactagtcgccacgctcccaccagcacggactgcgctctggggctagggagagtgggtgagcaggtggcagtacccacggctctcgctggagcggccgcgacccccgaccctggtccaatgtccctcgccggctgggcgcgcggggcgggaggtaccgcgctaggctgcccgggacgcccgccccgtccagtcagccggaaccgctcggcgccaat

SEQ ID NO: 15251 - RNA, 2311 nt, Homo sapiens
  source 1..2311: mol_type = other RNA
gctgggattacaggcatgagccactgcgccaggcctttgtgaggtgtcgttaatttgctctaccaaagacagcacaactggcacaagagctacaactggggccactatttgtgaatttgtgatagttcactctcatgctccaggatccatttggatttttcaggaggctgactattgaattagagatatgatttctttacttcttcaatgtctgtcacacttgggcaaaatggtatttttaatcaactttactgaggaataatttacatacaataaaatgcactcattttgagtgcatagtttgatgactttttgacaaacgtatgaatgaatgtaatcagtaccactgcaatcaaaatatagaacatttccatcaccccactatgttcttttgtgacccttttcaatttactattttgattgagggggaaagtttcaaaggattccacatagcttctctactgggaaggttcttaacctacagttctgagattcaatgtgggagttctactaactggcagttatgtccgctgcaataatatactgagggactagagagatgctcacccagtgggtttgtgggactggtggacctgaaccagaactcttccatttctcacctggtctccacgtatcctcctaagagggggccatgttaaaacagcaagtttcaatctcagtttctagctcattacttctattcaatagtcttcaaaatgtctgggacttgctcttccatcattgtttcataactgtatactatagtcattcacgattttgcagggtccttcatccttcagatccagccactccttcagttagtggcttccatgtctaaaaacttggttctatatattaaacaaaggactatgatttttttggggtggtcatccttaacatattgtcaaccattcttgacttcttttgattgtataaaataagcaaccctcttgctgactgcccatctctacagatttctgtaggtttggcactcttggatatcactttgacttgctattcatgatgataatggtgcctgctctgcattctatcatacagggccatcagggagcctggttctgaagcagcattgcctactgtcagccctagacaatagaagacgccactaagctttactgcaaggccatggcctgttaccagtacttttctcattatacaataaacaagtattctccaagcccacataacatagttggctggtgagttttctggccctatgtagaatatctactttagtatgcctacatctctgagtcttttttgttgttgttaaagccagtcaaatttagcagtggggggttgtatacctactttaatgacaccaatgttaataagttctcgtatacatctttgggtcttttgatccacccttcaattattggccatcataattctaatatttcaacgttacatggtatgggccatcattatctccaagcttcctagagcttaggtattagcaccatcttctgggaccctgtcagggttttaaattctttatatcagaacagtgctcatatcaataaattctcccttatccagatttatgttccaccttcatcacaccagcactttcaggctcctgtcccatacagcctctcctggctcctgcctacccatgttaggtgggtccagcagcaccttcaggacacaattctcctcctccctcagcaagcccagcacttctctagacacattacattgttcatcatgtgagttactggtctaaagccatgcagccaggtgtggtaccttctgagtggggtctttctgtgccaacttatcaacagaagttgctattgtaatgactgatctcttgtagtcttgatcggaaaatatattgagcactgaaacttgaggatgtttctttccatttttgtcaagaagagctgcttttgctatgttctcaacaatgtattttcttccggcttctgaaacgtttagtaaacaggcagccaaacggagccccactctggaagaagacatgatttttctgccccctgcgcacgcaccccaccggcacttggaggccgcaaggacgctcgccaggctgccgcaacgcgtgctggggccagaaccccgctgctgggattccctgcgcggtgccgactaggttcctgggtggagtgtcccaggaccacgtgggctgaaagggaacccgaagtgactcccggcctccccacaggtctcgcgggacgcagcagcggcgagggcgcggggttgtggcgcctgggagcgaggggcagccggcggctgcgctgccccggccgagctctcgaaccagcggccg

SEQ ID NO: 15252 - RNA, 874 nt, Homo sapiens
  source 1..874: mol_type = other RNA
gctgggattacaggcatgagccactgcgccatgccccgacatgttcttaaagagcagaaaaacatgtaacgcttagttcacttgaaagccttccacggaatacatttcagtgagtgacagacacaatgtttttgttccattagaagtattttattttaaagtacacttgaaattttaaatgtgtacaaattcagaggtttaaaaaacttcgaaagtcacagacacagaatttaggaagctgaaggctgagagtctcccttctcacttaatccatgctttattttgcattcctcacaggtaaggaggcagtgcctgttatgctgtggaccaaaaccagccccacggagctgatcttcaaaaaaatggaatttactctggcatactcctatgtatgatacctttccaaggccaaatcccaagagaccagcaagtgcaactttgggcaatgatccaaatctagaattagctgccaaataaccttggtagactagtccctgggtgacaagcatgcttacaagagaaaaaggcagagctctcttccagaaactttcttcctgacattctcgcataatctttgagatctctgctctgtggatgtgcagttttgattttggacaaaacaacaggctctgcttgcttggtggtggaaaatgggcatctttatcttggtttccacgagcagacgctgaagccatgatgactttgtgcttgctctccttccagttgtttatcctctgcttactccttgacccagtgtctgtgtggtctgggtcgcctccgaggccgagtccctcgttgccaagcccagcaggcctcgctcccccgtgactgcaccgccggcccgctccagcttcccgagtaccccacctgtctc

SEQ ID NO: 15253 - RNA, 777 nt, Homo sapiens
  source 1..777: mol_type = other RNA
gctgggattacaggcatgagccactgcgccatgccccgacatgttcttaaagagcagaaaaacatgtaacgcttagttcacttgaaagccttccacggaatacatttcagtgagtgacagacacaatgtttttgttccattagaagtattttattttaaagtacacttgaaattttaaatgtgtacaaattcagaggtttaaaaaacttcgaaagtcacagacacagaatttaggaagctgaaggctgagagtctcccttctcacttaatccatgctttattttgcattcctcacaggtaaggaggcagtgcctgttatgctgtggaccaaaaccagccccacggagctgatcttcaaaaaaatggaatttactctggcatactcctatgtatgatacctttccaaggccaaatcccaagagaccagcaagtgcaactttgggcaatgatccaaatctagaattagctgccaaataaccttggtagactagtccctgggtgacaagcatgcttacaagagaaaaaggcagagctgcttgcttggtggtggaaaatgggcatctttatcttggtttccacgagcagacgctgaagccatgatgactttgtgcttgctctccttccagttgtttatcctctgcttactccttgacccagtgtctgtgtggtctgggtcgcctccgaggccgagtccctcgttgccaagcccagcaggcctcgctcccccgtgactgcaccgccggcccgctccagcttcccgagtaccccacctgtctc

SEQ ID NO: 15254 - RNA, 779 nt, Homo sapiens
  source 1..779: mol_type = other RNA
gctgggattacaggcatgagccactgcgccatgccccgacatgttcttaaagagcagaaaaacatgtaacgcttagttcacttgaaagccttccacggaatacatttcagtgagtgacagacacaatgtttttgttccattagaagtattttattttaaagtacacttgaaattttaaatgtgtacaaattcagaggtttaaaaaacttcgaaagtcacagacacagaatttaggaagctgaaggctgagagtctcccttctcacttaatccatgctttattttgcattcctcacaggtaaggaggcagtgcgtgcaactttgggcaatgatccaaatctagaattagctgccaaataaccttggtagactagtccctgggtgacaagcatgcttacaagagaaaaaggcagagctctcttccagaaactttcttcctgacattctcgcataatctttgagatctctgctctgtggatgtgcagttttgattttggacaaaacaacaggctctgcttgcttggtggtggaaaatgggcatctttatcttggtttccacgagcagacgctgaagccatgatgactttgtgcttgctctccttccagttgtttatcctctgcttactccttgacccagtgtctaaggaaggtagaagagaatcactgtgtggtctgggtcgcctccgaggccgagtccctcgttgccaagcccagcaggcctcgctcccccgtgactgcaccgccggcccgctccagcttcccgagtaccccacctgtctc

SEQ ID NO: 15255 - RNA, 756 nt, Homo sapiens
  source 1..756: mol_type = other RNA
gctgggattacaggcatgagccactgcgccatgccccgacatgttcttaaagagcagaaaaacatgtaacgcttagttcacttgaaagccttccacggaatacatttcagtgagtgacagacacaatgtttttgttccattagaagtattttattttaaagtacacttgaaattttaaatgtgtacaaattcagaggtttaaaaaacttcgaaagtcacagacacagaatttaggaagctgaaggctgagagtctcccttctcacttaatccatgctttattttgcattcctcacaggtaaggaggcagtgcgtgcaactttgggcaatgatccaaatctagaattagctgccaaataaccttggtagactagtccctgggtgacaagcatgcttacaagagaaaaaggcagagctctcttccagaaactttcttcctgacattctcgcataatctttgagatctctgctctgtggatgtgcagttttgattttggacaaaacaacaggctctgcttgcttggtggtggaaaatgggcatctttatcttggtttccacgagcagacgctgaagccatgatgactttgtgcttgctctccttccagttgtttatcctctgcttactccttgacccagtgtctgtgtggtctgggtcgcctccgaggccgagtccctcgttgccaagcccagcaggcctcgctcccccgtgactgcaccgccggcccgctccagcttcccgagtaccccacctgtctc

SEQ ID NO: 15256 - RNA, 2386 nt, Homo sapiens
  source 1..2386: mol_type = other RNA
gctgggattacaggcatgagccactgcgcccagatggttccatatttttccaattgcaaattgtgctgctataaacacgcatgagcaagtatctttttcgtataatgacttattttcctctgggtagatgccccgtagtgggattgctggatcaaatggtagatctactttttgttctttaaggatccacaatgttttccatcgtggttgtactagtgtttgtactagtttacatttcatggaaaaactttctatagaagaaaatgtgaactacagagaaaaaaaaatcaaaatcacaggaagaagatagcaatctacttcattcctggaattgtctgaaaaagtcgtgtaaaatttgtggagatttaagtatatggagaaaaacacttattcattgtaagtaaaataagattgtatttcagcttcatcttgtgtatacttaggagtaatagaaaagagacaaatggggagagaataaaagaaatataggaagaggaaaagagaaaagaatcaggaaattggaagtgaaataattccacacatacttattgaagtctatttaaacaatgcttaaaaatatatggcctcttagaattatacgtttaaaatgaactttgtcgctatgggatttggggcattataacaggaagtgagatgtttgaagacagggtttttgagctctctgggtattaactccttaagtgaaagatgctctgagtgcacaatagacttgtgctgtgttctttaattgatggagatgctacatctcatgtcctcatcatccacagagcctccagatcctggccagaagtctcctcagagcccccttcatatctttatttctcagggtgtaggtgaagggattgagagtgggggtgattatggaatagaagagagaaataaatttgccctgctcttgggagtagctggaagggggctgcagatacatgtaaatcgcaggtaggtagaagagggagacgatcatcaggtgggaggaacacgtcccaaaggccttgtgtcgtcccttggaggactggatcctgagcactgcccgggcaataaagccataggagagaaggatgagagccaggggcaccaacacgaagaaggccaccagcacagccagtatggtgtcattcacagcggtgtcagcacacgacagcttgatcacggccggcacctcacagaaaaagttgttcagcacctgccgcccgcagaatggcaattgcaccgtcaggaccacctgcacgaaggagttgccgaagccactgagccaggccagagccacgagctgctgacagagagcacggtgcatgagaacggcatagtgcaggggcttgcagatggccacgtagcggtccagggccatggcggccaggacgatgcactccgtgcatcccagccagtggaagactgcatattgcacagtgcagcctccatagctgatggtcttctgggaactgcccatgttgaccagcatctgagggactgtcgtggtggtgtagcagaggtccaggaaggacaggtgactgaggaagatgtacatggggctgtggagttgaggatccacccgggatgccaggatgatggcgacgttccccaacatggccagcacataggacagcaggaggaccacaaagagagggagttccagccacggcctctgtggagacgctgggatgcggaagggtcagaaccaggagccccagtagcagcctctgtgtctttgctctccttcctactcagtggccgcaactaaaccatttaatattcctgaacttctgcatctcacgaatgacaattatgttccaggtagagcgaagcgtgctgcagctcccatcaccgtcagagtgtttgatttctctctacatccacatcgacaaggaattgtccaccttcttaggctgctgattgtatcatgttcacgctgaattcccgcagtttcttctgggggctgctggcaggctaggctgtgaacacgcaggctgtgatacacccttagatatatatcattccctccagggttcctggctcctacagaagacttgctttaggactgaaggctatattgcagtctgtgttggccttagtcgcggagggacatttaaggatggacttactagaaatgctcttcatattccaggaacacacagcacatttcctctgatgggctgctgggaccttaccatttactggaacccaaccctctgagcaagtctgagagattattctcagtctagaaggagtctgctgtccgttgcaacaggcttgctggggagactcagggtttcccggactctcccttggcagtacgtgaggtcggtggaactgccttaaccttagtcccccagagtgcctataggtaccttgacatggtggaggttac

SEQ ID NO: 15257 - RNA, 752 nt, Homo sapiens
  source 1..752: mol_type = other RNA
gctgggattacaggcatgagccactgcgcccagcaagggcctcagtttcttcatgtcaaatgccacacatgcaggacagacattttgttagcaccttctggttctatcattttcgtaatctgtaacttcagttggttggtctggtctcagaatcacacattggtccagaattacacttgccctgctctgaagaagaatgccacctgcttgtcagctttggagtcaacagccctgaggactcaagtccccttttgacagagtggctctggacaagtcacttgcctttccttctccatctgatatgttctgtcctcaggtgctatctggcttgaaccaagccttgacttttcaaggagaggaacagctgggcctcagtggagaatttcaggaattttctgccttgctcactggttttgccctgccattgtcctggggtgggctcccagaatacccttgggctccttaggtggggcggggcaaggtggatactgcctggggcggagggagggactgtgctgtgctctgttcccttctgacttactgtttgtttggggcgtctggacgagggctacaaacagttcctccctttgtttccacggccttgcagaatgtgtgcttccctcaaaagggcataaaggccccctttcttctgctctcctgcgccacggggggttgttctgcagggctcgggtctacaagctgaggccagccccaagcgctgactgtagcagctccatccgctcccacagcct

SEQ ID NO: 15258 - RNA, 1723 nt, Homo sapiens
  source 1..1723: mol_type = other RNA
gctgggattacaggcatgagccactgcgcccagcagtactaagataaatttaaccttctcattttaaagatgaggaaattaaaccaggacctaatgaaggaaaatggcttatccaaggctacgtggttactgctagagccaggataagaatgtgggttgtctgaatattgtgtttctttcactctttcgtattaactattaggcaaactttctgtctgcctattaaaattcaagtctgaatgcccttcttaggccccaatcaggatatccaaaagccacttgcacaataattcgaccgtgcacttgttaagttgtgaagatgaacgaagtagcaactcaaggaaacgtcaaccaatggtatgatttcacattaagttgtctaatttgctttgtggtggtgggttcatcccggtactacccataaacgaatcagtaaatgagacttagtttccaaccttacttcccgactagacaactgcatgaaaaattggatagcgaattatgagtccaagttctatagctggcatagtcctcatgctttagccccagcctctgagcttagcagaagacattttgggtccttatatattgctagtaggattgtataattcttgactgtgttgcagaatcttacaggactacaaaacttaccatgatgtgtcttataaggaagacttgccaggcaaattttcgggcaagccagcaaaatagttaaagtaagagtaaagaggaacacgtgaatgatggggagttggtctaggaaaatattgtgaggaaaataaatgaaattctatggttagcccaaatagacaaagatagcttcttcaaccctaagatctatatcagacagattcaatagtaaagattattagcctaaagtttagtctcccttgaaattgtacatagaatgtttgtatataagccatatagtcatcatctattcactgtgtctatgatattgagaagcagcaaaattatgcaataatatagactttgtattttaagtgctagaaaatgagataaatgttatcagtttgggtgaaaaagtagagagtaggggtaaaagctggacattgcaaaaggattggtttaagaaatactgtctaagggttagctgtcaatggttggagaagaaggagatcctccttcctctcacccatacattttttcttctttcctctttttcaatgatcacagaccattgggtctctgcaaatccacattttcacagggaggaagtcggaagtaattggagcgacggagtctcctagggggcagaccagccatctgacggcaaagctcatccaagtcatctgtggaaggtgcaatatcagccaaaacagccaaaactgtttcatctgtagcgggatcattcaccagattaggatcttctgtgaatgtttctggagtcgcttgagtcacatcgtctcctcgttgactattgacccccaggggtatccagtcagaggtgatgatgaatgcagcaagaaacagcagcaccttgggtcccaagagcgacatattgtctatggtgttctgctctttccaccgagtcctttggctgctgaatgtgtctctctcctcttacgctgttcctactttggctggcgaataagatgaacagagccactccctggaaaggacttcagatttggcctccgctgaaacaatgagatgagggagagcaagaaagccaggctaggcgtagaatgtgtgttacaat

SEQ ID NO: 15259 - RNA, 1954 nt, Homo sapiens
  source 1..1954: mol_type = other RNA
gctgggattacaggcatgagccactgcgcccagcagtactaagataaatttaaccttctcattttaaagatgaggaaattaaaccaggacctaatgaaggaaaatggcttatccaaggctacgtggttactgctagagccaggataagaatgtgggttgtctgaatattgtgtttctttcactctttcgtattaactattaggcaaactttctgtctgcctattaaaattcaagtctgaatgcccttcttaggccccaatcaggatatccaaaagccacttgcacaataattcgaccgtgcacttgttaagttgtgaagatgaacgaagtagcaactcaaggaaacgtcaaccaatggtatgatttcacattaagttgtctaatttgctttgtggtggtgggttcatcccggtactacccataaacgaatcagtaaatgagacttagtttccaaccttacttcccgactagacaactgcatgaaaaattggatagcgaattatgagtccaagttctatagctggcatagtcctcatgctttagccccagcctctgagcttagcagaagacattttgggtccttatatattgctagtaggattgtataattcttgactgtgttgcagaatcttacaggactacaaaacttaccatgatgtgtcttataaggaagacttgccaggcaaattttcgggcaagccagcaaaatagttaaagtaagagtaaagaggaacacgtgaatgatggggagttggtctaggaaaatattgtgaggaaaataaatgaaattctatggttagcccaaatagacaaagatagcttcttcaaccctaagatctatatcagacagattcaatagtaaagattattagcctaaagtttagtctcccttgaaattgtacatagaatgtttgtatataagccatatagtcatcatctattcactgtgtctatgatattgagaagcagcaaaattatgcaataatatagactttgtattttaagtgctagaaaatgagataaatgttatcagtttgggtgaaaaagtagagagtaggggtaaaagctggacattgcaaaaggattggtttaagaaatactgtctaagggttagctgtcaatggttggagaagaaggagatcctccttcctctcacccatacattttttcttctttcctctttttcaatgatcacagaccattgggtctctgcaaatccacattttcacagggaggaagtcggaagtaattggagcgacggagtctcctagggggcagaccagccatctgacggcaaagctcatctagcacaggtgagcagtaaatgttagtttcctttatatatccagctgccaattcttctaatcatggatctttcatagcttcgtgttccttacagacaagacgagagcagatctccttgttgacgatgtacatacgtcgtaaactggtgaagcataactgatgaatgcattgtttaaccggccgatgcacagagtagagccttgtgcaggtaaatttctcatcccagcactccaagtcatctgtggaaggtgcaatatcagccaaaacagccaaaactgtttcatctgtagcgggatcattcaccagattaggatcttctgtgaatgtttctggagtcgcttgagtcacatcgtctcctcgttgactattgacccccaggggtatccagtcagaggtgatgatgaatgcagcaagaaacagcagcaccttgggtcccaagagcgacatattgtctatggtgttctgctctttccaccgagtcctttggctgctgaatgtgtctctctcctcttacgctgttcctactttggctggcgaataagatgaacagagccactccctggaaaggacttcagatttggcctccgctgaaacaatgagatgagggagagcaagaaagccaggctaggcgtagaatgtgtgttacaat

SEQ ID NO: 15260 - RNA, 1984 nt, Homo sapiens
  source 1..1984: mol_type = other RNA
gctgggattacaggcatgagccactgcgcccagcagtactaagataaatttaaccttctcattttaaagatgaggaaattaaaccaggacctaatgaaggaaaatggcttatccaaggctacgtggttactgctagagccaggataagaatgtgggttgtctgaatattgtgtttctttcactctttcgtattaactattaggcaaactttctgtctgcctattaaaattcaagtctgaatgcccttcttaggccccaatcaggatatccaaaagccacttgcacaataattcgaccgtgcacttgttaagttgtgaagatgaacgaagtagcaactcaaggaaacgtcaaccaatggtatgatttcacattaagttgtctaatttgctttgtggtggtgggttcatcccggtactacccataaacgaatcagtaaatgagacttagtttccaaccttacttcccgactagacaactgcatgaaaaattggatagcgaattatgagtccaagttctatagctggcatagtcctcatgctttagccccagcctctgagcttagcagaagacattttgggtccttatatattgctagtaggattgtataattcttgactgtgttgcagaatcttacaggactacaaaacttaccatgatgtgtcttataaggaagacttgccaggcaaattttcgggcaagccagcaaaatagttaaagtaagagtaaagaggaacacgtgaatgatggggagttggtctaggaaaatattgtgaggaaaataaatgaaattctatggttagcccaaatagacaaagatagcttcttcaaccctaagatctatatcagacagattcaatagtaaagattattagcctaaagtttagtctcccttgaaattgtacatagaatgtttgtatataagccatatagtcatcatctattcactgtgtctatgatattgagaagcagcaaaattatgcaataatatagactttgtattttaagtgctagaaaatgagataaatgttatcagtttgggtgaaaaagtagagagtaggggtaaaagctggacattgcaaaaggattggtttaagaaatactgtctaagggttagctgtcaatggttggagaagaaggagatcctccttcctctcacccatacattttttcttctttcctctttttcaatgatcacagaccattgggtctctgcaaatccacattttcacagggaggaagtcggaagtaattggagcgacggagtctcctagggggcagaccagccatctgacggcaaagctcatctagcacaggtgagcagtaaatgttagtttcctttatatatccagctgccaattcttctaatcatggatctttcatagcttcgtgttccttacagacaagacgagagcagatctccttgttgacgatgtacatacgtcgtaaactggtgaagcataactgatgaatgcattgtttaaccggccgatgcacagagtagagccttgtgcaggtaaatttctcatcccagcactctgcagtggtatttttttcactgagggaggccaagtcatctgtggaaggtgcaatatcagccaaaacagccaaaactgtttcatctgtagcgggatcattcaccagattaggatcttctgtgaatgtttctggagtcgcttgagtcacatcgtctcctcgttgactattgacccccaggggtatccagtcagaggtgatgatgaatgcagcaagaaacagcagcaccttgggtcccaagagcgacatattgtctatggtgttctgctctttccaccgagtcctttggctgctgaatgtgtctctctcctcttacgctgttcctactttggctggcgaataagatgaacagagccactccctggaaaggacttcagatttggcctccgctgaaacaatgagatgagggagagcaagaaagccaggctaggcgtagaatgtgtgttacaat

SEQ ID NO: 15261 - RNA, 1849 nt, Homo sapiens
  source 1..1849: mol_type = other RNA
gctgggattacaggcatgagccactgcgcccagcagtactaagataaatttaaccttctcattttaaagatgaggaaattaaaccaggacctaatgaaggaaaatggcttatccaaggctacgtggttactgctagagccaggataagaatgtgggttgtctgaatattgtgtttctttcactctttcgtattaactattaggcaaactttctgtctgcctattaaaattcaagtctgaatgcccttcttaggccccaatcaggatatccaaaagccacttgcacaataattcgaccgtgcacttgttaagttgtgaagatgaacgaagtagcaactcaaggaaacgtcaaccaatggtatgatttcacattaagttgtctaatttgctttgtggtggtgggttcatcccggtactacccataaacgaatcagtaaatgagacttagtttccaaccttacttcccgactagacaactgcatgaaaaattggatagcgaattatgagtccaagttctatagctggcatagtcctcatgctttagccccagcctctgagcttagcagaagacattttgggtccttatatattgctagtaggattgtataattcttgactgtgttgcagaatcttacaggactacaaaacttaccatgatgtgtcttataaggaagacttgccaggcaaattttcgggcaagccagcaaaatagttaaagtaagagtaaagaggaacacgtgaatgatggggagttggtctaggaaaatattgtgaggaaaataaatgaaattctatggttagcccaaatagacaaagatagcttcttcaaccctaagatctatatcagacagattcaatagtaaagattattagcctaaagtttagtctcccttgaaattgtacatagaatgtttgtatataagccatatagtcatcatctattcactgtgtctatgatattgagaagcagcaaaattatgcaataatatagactttgtattttaagtgctagaaaatgagataaatgttatcagtttgggtgaaaaagtagagagtaggggtaaaagctggacattgcaaaaggattggtttaagaaatactgtctaagggttagctgtcaatggttggagaagaaggagatcctccttcctctcacccatacattttttcttctttcctctttttcaatgatcacagaccattgggtctctgcaaatccacattttcacagggaggaagtcggaagtaattggagcgacggagtctcctagggggcagaccagccatctgacggcaaagctcatctttcatagcttcgtgttccttacagacaagacgagagcagatctccttgttgacgatgtacatacgtcgtaaactggtgaagcataactgatgaatgcattgtttaaccggccgatgcacagagtagagccttgtgcaggtaaatttctcatcccagcactccaagtcatctgtggaaggtgcaatatcagccaaaacagccaaaactgtttcatctgtagcgggatcattcaccagattaggatcttctgtgaatgtttctggagtcgcttgagtcacatcgtcagaggtgatgatgaatgcagcaagaaacagcagcaccttgggtcccaagagcgacatattgtctatggtgttctgctctttccaccgagtcctttggctgctgaatgtgtctctctcctcttacgctgttcctactttggctggcgaataagatgaacagagccactccctggaaaggacttcagatttggcctccgctgaaacaatgagatgagggagagcaagaaagccaggctaggcgtagaatgtgtgttacaat

SEQ ID NO: 15262 - RNA, 1885 nt, Homo sapiens
  source 1..1885: mol_type = other RNA
gctgggattacaggcatgagccactgcgcccagcagtactaagataaatttaaccttctcattttaaagatgaggaaattaaaccaggacctaatgaaggaaaatggcttatccaaggctacgtggttactgctagagccaggataagaatgtgggttgtctgaatattgtgtttctttcactctttcgtattaactattaggcaaactttctgtctgcctattaaaattcaagtctgaatgcccttcttaggccccaatcaggatatccaaaagccacttgcacaataattcgaccgtgcacttgttaagttgtgaagatgaacgaagtagcaactcaaggaaacgtcaaccaatggtatgatttcacattaagttgtctaatttgctttgtggtggtgggttcatcccggtactacccataaacgaatcagtaaatgagacttagtttccaaccttacttcccgactagacaactgcatgaaaaattggatagcgaattatgagtccaagttctatagctggcatagtcctcatgctttagccccagcctctgagcttagcagaagacattttgggtccttatatattgctagtaggattgtataattcttgactgtgttgcagaatcttacaggactacaaaacttaccatgatgtgtcttataaggaagacttgccaggcaaattttcgggcaagccagcaaaatagttaaagtaagagtaaagaggaacacgtgaatgatggggagttggtctaggaaaatattgtgaggaaaataaatgaaattctatggttagcccaaatagacaaagatagcttcttcaaccctaagatctatatcagacagattcaatagtaaagattattagcctaaagtttagtctcccttgaaattgtacatagaatgtttgtatataagccatatagtcatcatctattcactgtgtctatgatattgagaagcagcaaaattatgcaataatatagactttgtattttaagtgctagaaaatgagataaatgttatcagtttgggtgaaaaagtagagagtaggggtaaaagctggacattgcaaaaggattggtttaagaaatactgtctaagggttagctgtcaatggttggagaagaaggagatcctccttcctctcacccatacattttttcttctttcctctttttcaatgatcacagaccattgggtctctgcaaatccacattttcacagggaggaagtcggaagtaattggagcgacggagtctcctagggggcagaccagccatctgacggcaaagctcatctttcatagcttcgtgttccttacagacaagacgagagcagatctccttgttgacgatgtacatacgtcgtaaactggtgaagcataactgatgaatgcattgtttaaccggccgatgcacagagtagagccttgtgcaggtaaatttctcatcccagcactccaagtcatctgtggaaggtgcaatatcagccaaaacagccaaaactgtttcatctgtagcgggatcattcaccagattaggatcttctgtgaatgtttctggagtcgcttgagtcacatcgtctcctcgttgactattgacccccaggggtatccagtcagaggtgatgatgaatgcagcaagaaacagcagcaccttgggtcccaagagcgacatattgtctatggtgttctgctctttccaccgagtcctttggctgctgaatgtgtctctctcctcttacgctgttcctactttggctggcgaataagatgaacagagccactccctggaaaggacttcagatttggcctccgctgaaacaatgagatgagggagagcaagaaagccaggctaggcgtagaatgtgtgttacaat

SEQ ID NO: 15263 - RNA, 1915 nt, Homo sapiens
  source 1..1915: mol_type = other RNA
gctgggattacaggcatgagccactgcgcccagcagtactaagataaatttaaccttctcattttaaagatgaggaaattaaaccaggacctaatgaaggaaaatggcttatccaaggctacgtggttactgctagagccaggataagaatgtgggttgtctgaatattgtgtttctttcactctttcgtattaactattaggcaaactttctgtctgcctattaaaattcaagtctgaatgcccttcttaggccccaatcaggatatccaaaagccacttgcacaataattcgaccgtgcacttgttaagttgtgaagatgaacgaagtagcaactcaaggaaacgtcaaccaatggtatgatttcacattaagttgtctaatttgctttgtggtggtgggttcatcccggtactacccataaacgaatcagtaaatgagacttagtttccaaccttacttcccgactagacaactgcatgaaaaattggatagcgaattatgagtccaagttctatagctggcatagtcctcatgctttagccccagcctctgagcttagcagaagacattttgggtccttatatattgctagtaggattgtataattcttgactgtgttgcagaatcttacaggactacaaaacttaccatgatgtgtcttataaggaagacttgccaggcaaattttcgggcaagccagcaaaatagttaaagtaagagtaaagaggaacacgtgaatgatggggagttggtctaggaaaatattgtgaggaaaataaatgaaattctatggttagcccaaatagacaaagatagcttcttcaaccctaagatctatatcagacagattcaatagtaaagattattagcctaaagtttagtctcccttgaaattgtacatagaatgtttgtatataagccatatagtcatcatctattcactgtgtctatgatattgagaagcagcaaaattatgcaataatatagactttgtattttaagtgctagaaaatgagataaatgttatcagtttgggtgaaaaagtagagagtaggggtaaaagctggacattgcaaaaggattggtttaagaaatactgtctaagggttagctgtcaatggttggagaagaaggagatcctccttcctctcacccatacattttttcttctttcctctttttcaatgatcacagaccattgggtctctgcaaatccacattttcacagggaggaagtcggaagtaattggagcgacggagtctcctagggggcagaccagccatctgacggcaaagctcatctttcatagcttcgtgttccttacagacaagacgagagcagatctccttgttgacgatgtacatacgtcgtaaactggtgaagcataactgatgaatgcattgtttaaccggccgatgcacagagtagagccttgtgcaggtaaatttctcatcccagcactctgcagtggtatttttttcactgagggaggccaagtcatctgtggaaggtgcaatatcagccaaaacagccaaaactgtttcatctgtagcgggatcattcaccagattaggatcttctgtgaatgtttctggagtcgcttgagtcacatcgtctcctcgttgactattgacccccaggggtatccagtcagaggtgatgatgaatgcagcaagaaacagcagcaccttgggtcccaagagcgacatattgtctatggtgttctgctctttccaccgagtcctttggctgctgaatgtgtctctctcctcttacgctgttcctactttggctggcgaataagatgaacagagccactccctggaaaggacttcagatttggcctccgctgaaacaatgagatgagggagagcaagaaagccaggctaggcgtagaatgtgtgttacaat

SEQ ID NO: 15264 - RNA, 1840 nt, Homo sapiens
  source 1..1840: mol_type = other RNA
gctgggattacaggcatgagccactgcgcccagcagtactaagataaatttaaccttctcattttaaagatgaggaaattaaaccaggacctaatgaaggaaaatggcttatccaaggctacgtggttactgctagagccaggataagaatgtgggttgtctgaatattgtgtttctttcactctttcgtattaactattaggcaaactttctgtctgcctattaaaattcaagtctgaatgcccttcttaggccccaatcaggatatccaaaagccacttgcacaataattcgaccgtgcacttgttaagttgtgaagatgaacgaagtagcaactcaaggaaacgtcaaccaatggtatgatttcacattaagttgtctaatttgctttgtggtggtgggttcatcccggtactacccataaacgaatcagtaaatgagacttagtttccaaccttacttcccgactagacaactgcatgaaaaattggatagcgaattatgagtccaagttctatagctggcatagtcctcatgctttagccccagcctctgagcttagcagaagacattttgggtccttatatattgctagtaggattgtataattcttgactgtgttgcagaatcttacaggactacaaaacttaccatgatgtgtcttataaggaagacttgccaggcaaattttcgggcaagccagcaaaatagttaaagtaagagtaaagaggaacacgtgaatgatggggagttggtctaggaaaatattgtgaggaaaataaatgaaattctatggttagcccaaatagacaaagatagcttcttcaaccctaagatctatatcagacagattcaatagtaaagattattagcctaaagtttagtctcccttgaaattgtacatagaatgtttgtatataagccatatagtcatcatctattcactgtgtctatgatattgagaagcagcaaaattatgcaataatatagactttgtattttaagtgctagaaaatgagataaatgttatcagtttgggtgaaaaagtagagagtaggggtaaaagctggacattgcaaaaggattggtttaagaaatactgtctaagggttagctgtcaatggttggagaagaaggagatcctccttcctctcacccatacattttttcttctttcctctttttcaatgatcacagaccattgggtctctgcaaatccacattttcacagggaggaagtcggaagtaattggagcgacggagtctcctagggggcagaccagccatctgacggcaaagctcatctttcatagcttcgtgttccttacagacaagacgagagcagatctccttgttgacgatgtacatacgtcgtaaactggtgaagcataactgatgaatgcattgtttaaccggccgatgcacagagtagagccttgtgcaggtaaatttctcatcccagcactctgtttcatctgtagcgggatcattcaccagattaggatcttctgtgaatgtttctggagtcgcttgagtcacatcgtctcctcgttgactattgacccccaggggtatccagtcagaggtgatgatgaatgcagcaagaaacagcagcaccttgggtcccaagagcgacatattgtctatggtgttctgctctttccaccgagtcctttggctgctgaatgtgtctctctcctcttacgctgttcctactttggctggcgaataagatgaacagagccactccctggaaaggacttcagatttggcctccgctgaaacaatgagatgagggagagcaagaaagccaggctaggcgtagaatgtgtgttacaat

SEQ ID NO: 15265 - RNA, 13196 nt, Homo sapiens
  source 1..13196: mol_type = other RNA
gctgggattacaggcatgagccactgcgcccagccaaacttatctttgtatgtttgttataggcaaaagtaccccaaggttaaggctcagcccaagaggtcaagtgggttcaggaaagaattcaagagcatgctgacagaataaagtgaaagcaagttcattaagaaagtaaaggaataaaagaatggctaccccataggaagagtagccctgatgggctgctgactggctatatttatggttgcttcttgactatacgctaaacaagaggtggcttattcatgagttttccaggaaagaagtggggaggtctggaccttttagaccatacagggtaacttctgaaagttgctatggcagttgtaaactatcatggtgctgtagaagtttcttttagcgtgctaatgtattataattaccatagaatgggcagcaaaggtaaccagaggtctcttctgtcaccatcatggttttggctggtttgggttggcctttctaccacatcctgtcttatcagcagggtcttacagggtcttgtggtcttgggaaaccagtcctgccaaactcctctcattcagtgtaatcactatcaaaattccagaggccctttttacataaatttgcaagtgaatcctaacagttatatgaaaatttagggaaaggtaaacccaatacagccctaacaattttgaaaaagaacaggccagttgcagtggctcacccctcagcactttgggaggtggaggtgggaggattgtttgaggccaggagtttgagaccagcctgggcaacatagcaaggcctcatctctacaaaagaaaaaagaagaacaacaacaacaacaaagttagaggactacatttctggattccaaaacttactacgaagttacaataatcaagacagtgtggtactaccataagatagagcaacagaattgagtccagaaataaacccttatagttagttgatttgtgataagtataaaataattctatagggaaaaaatagtattttcaataagtaatgctaagacaagtgaacatttatgtgcaaaagaatgaggctggatgcttatctcgcactgcatacacaaaaataactcaaaatgggtcaaagagctaaaatcataaaactttagaagaaaacataggggtaacacctcataggcaattgatttagacaatggttttttaggtatgacaccaaaagcataagcaataacataaaaaacagaaatcaagtgaacttcatcaaaatttaaaacttgtactgtatagtatccagaaagtgagaagacaatccatggaatgggagaatatattcacaaagattgtacctgataagaaactagtatccagaatattaaaaagaatgcttacaactcaacaataaaaagacaacccaccgggtgtggtggctcacgcctgtaatcctagcattttgggaggccgaggcaggcagatcacctgagttcaggagttcaagaccagcctggccaacatggcgaaaccctgtctctactaaaaatacaaaaattagccaggcgtgatggtgggtgcctgtaatcccagttactagggaggccgaggcaggagagtcgcttgaactcaggaggtggaggttgcagtgagccgagattgcaccactgcactccaacctgggcgacagagtgagattccatctcagaaaaataaaataaaataacgcagttttaaaatgagaaaggacttgaggccaggcacagtagctaatgtctgtaatgccagcactttgggaagccaaggcagtcagatcacctgaggccaggagttcgagaccagcctggccaacatggtgaaaccctgtctttactaaaaatacaaaaattggctgggcgcggtggctcacgcctgtaatcccagcactttgggaggccaaggcaggcggatcacgaggtcaggagatagagaccatcctggctaacacggtgaaaccctgtctctactaaaaatacaaaaaattagccgggcgtggtggagggcggctgtagtcccagatacttgggaggctgaggcaggagaatggcatgaacccaggaggcggagcttgcagtgagctgagattgcaccactgcactccagcctgggccacagagcgagactccgtctcaaaaaacaatacaaaaattagttgggcatggtggcgagctcctgtaaacccagctactcccaactactagggaggctgaggcaggagaatggcttgaacccagaaggcagaggttacagtgaatcaagataacgccactgcactccaccctgggcgacagagtgagactccgtctcaaaaacaaaaaaataaaaaaaacctcatacactgctggtgggaatataaaatgatgctactactttgaaaagcagtttggcagttcctcaaaaggctaaacatagagttactatatgatgagcactctcacttctaaggtatatgcccagaagaactgaaaacatatatccatataaaaattcatatacgaatattcatagcagcatcatccataatagcaaaaaagtggaaacagtctaaatttcgatcaactgatgaataaactaaatgcggtatatccacacaatagggtattattcagccataaaatgtaatgaagcactggtacactctatagcatagatgaaccttgaaacatgctaagtgaaggaagtcagacacgaaaggccacatgtttatttttataaaatatctagaacaggcaaatcatagagacagaaaatggattattgtttctagaggctgggggaagaggaggattagagtggcagctcactggtatggagtttctaggtagatggaaatgttctggaattagatagtggtgatgattgcacaactctgtaaatatactaaaatccactgcatcatttactttaaaggggcaaattttatggcttgtgaattacatttcaataaaaagaagatgaggaaacctaggatatgtcacaatcccatgccacaaactacttacacttccaatataaaaactatatcaacaatagtttacatcacgttcattgcttgctaaagtaaggtcatgaatgtatcaaaatattttataaaagttaaaatttaggagatccatcatttctcttttcaatccatcactgattcattcaatatatatttatgtgtatgccaggctcttcatcaggtaaagtgtttaggagagatataaagataaaactgatgagaattctgcacttgagctacagcatactttccaagaattacagcatgagatataaaatgaaaagaaggcttggaggagattcacacgaaatagtactgttcaggagagggggcgataattccaatggaagagataactgacttcatggaggatagaaggagatggtatttgaactgcccttgaagtatggttatattttggggatgtggagatgtggggtagggtgatatgctggggttccagatggtccagaaatatacaatcaccagaaccaaagatccagaggtaggagatatgagctgttcaatttggctgagctaacagtgtttggagtgggatcttgaagaagctgaaaatgaagataccaactagacagtcagagaaagacttccaatgtttgactgaactgcaattttattgtgtatgcattgaagaatctttttttttttttttgtattctctaaagatttttaaaatattttaagttctggatacaagtgcaggatgtgcgggtttgttacataggtaaacgtgtcccatggtggtttgctgcacctatcaacctatcacctaggtattaagccccacatgcattagctagttatcctgatgctctccccgctacggcccctgcatcaggccccagtgtgtgttgatctcatccctgtgtccgtgtgttctcattgttcagcttccgcttacaagtgagaacatgtggtgtttggtttcctgctcctctgttagtttgctgaggataatggcttccagcttcatccatgtccctgcaaaggacatgatctcattccttttttaaaaaaaaaaacaaaattatttccataggtgtttggggaacaggtggtatctggttacatgcgtaagtaattaagtggttacttgtgagattctggtgcacccatcacctgagcagtatacactgaacccaatttgtattcttttatccttcacccccctcccaccctttcccctaagtccccaaagtccattgtatccttcttatgcctttgcatcctcatagcttatctcccacttatgagtgagaacatacaatgtttggttttccattcctcagttacttcctttagagtaatagtctccaggttgctgtgaatgtcattaattcattcctttttatggctgagtagtgtttaggtgaggttatttgtaagtaattaatattgagtaaataagattcatccatagtggcaaagccacataacttctaagtatcttaaactatatctaaatggtaccaaaacatgcagtcaattctaaaagctcagctaatgatatttcataatataggaaaatattcacaacatatttttgtgtaaaaaaaagcagacttcaaaatggaatatgcattatgattccaatcatgtaaaagctatacatgaacacatacaaagattaacagatataaacaaatggaagaatgaatggagagatagatgatagacagattgagtggtggtggagaataacagatttaaaaagaaattgtgcctttctatattttcaaaaccatttaaataagtattacctttggagttagaaaatgatatgtattttaaatccataattcaactacttatctatatgatgtcaaactggattaggctgaattatcagcaagtgaataaaacagttccttcatccatggagaaacatccatttatgacattcttggaattcctcttgttagaattctttatgaatttaaaatagaaacatggccagactcaagatttcaatacaaacattactttttcacgttcagtaataaccaattaaaagaattaatgaaaaatctgattcactgtatcaccaaaagctgtaatggctgcactgcacagtattccatggtgtatatgtaccacattttctttatccagtctatctttgatgggcatttgctattgtgtctttgctattgtgaagagtgctgcaatgaacaaaaatgtgcatgtatctttataataaaatggtttatattcctttgggtatatacccagtaatgggattgctgggacaaatagtatttctagttctagatctttgaggaatagccacacacacttccacaacggttgaactaatttacattcccaccaacaatgtaaaagtgttcctacttctccacagcctcgccagcatctgttgttttttgactttttaataatcaccattctgaccggcatgagatggtatctcattgtggttctcctttgcatttctctaatgatcagtaaggttgagcttttttttatatgtttgttggccacataaatgtcttcttttgagaagtgtctgttcatgtcctttgtccactttttgatggggttgtttttttccttgtaaatttgttttaagttccttgtaggttctggatattagacctttgtcagatggatagattgcaaaaatgttctcccattctgtaggttgcctgttcactctaatgatagtttcttttgctgtgcaggagctctttagtttaattagatcccatttgtaatttttgcttttgttgcaattgcttttgatgtttttgtcatgaaacctttgcttgtgcctatgtcttgaatggtattaaatagattttcttctagggtttttatagttttaggttttacattaagtctttaatcttgagttaatttttgtataaggtgtaaggaaggggtcagtttcaattttctgcatatggctagccagttttcccagcaccatttattaaatagggaatcttttccccattgcttgtttttgtcaggtttgtcgatgatcagatggctgtagatgtgtggtcttctttctctggtctctattctgttccattggtctatgtgtctgtttttgtaccagtaccatgccattttggctactgtagccttgcagtatactttgaagttgggtagtgtgatgcttccagctttgttctttttgcttattgttgtcttggttatacgggctcttttttggttccatttgaattttaaagtagtttttttctaattctgtgaagaatgtcaatagtagtttaatgggaatagcaatgaacctataaattactttgggtagtatggccattttcatgatattgattcttcctatccacgagaatggaatgttttttcatttgtgtcctctcttatttccttgagcagtggtttgtagttctccttgaagagatccttcacatcttattagctgtattcctaggtattttattctctttctagcaactgtgaatgggagttcattcatgatttggctctctgcttgtgtattgttggtgtatagaatgcttgtgatttctgcacattgattttgtatcctgagactttgctgaagttgcttatcagcttaaggaacttttgggtggagataatggggttttctagatatagtatcatgtcatctgcaaacacagttttacttcctcttttcctatttgaataccccttatttgtttctcttgcctgattttcttggccagaacttccaatactatgttaaataggagtggtgagacggcatccctgtcttgtgccagttttcaaggggaatgcttccagcttttgcccattcagtatgataatggctgtgggtttgtcataaatggttattattttgagatattttccatcaatacctagtttattgagagtttttaacatgaagcaacgttgaattttattgaaggccttttctgtatctattgagataatcatgtggtttttgtctttagttctgtttatgtgatgaattatgtttcttgatttgcgtatgttgaaccagccttgcatcccagggatgaagccaacattccaaacattttatttattatttatttatttatttatttttgagacagagtctcgcactgtcgcccaggctggagtgcagtggcaagatctcagctcgctgcaagctccacctcccaggttcatgccgttctcttgcctcggcctcccaaatagcagggactacaggcgaccgccacaacgcctggctaattttttgtatttttagtagagacggggttttacatgttagccaggatggtcttgatctcctgacctcgtgatccgcccgccttggcctcccaaagggctgggattataggcgtgagccaccgcacccggcctccaaacattttaatctcataacaatgcatcacttgggttaactaggttgagataaatataaactgtcaattttttttcccctcacataaaagtccagaggtaggtaattagggctgacacagtgattccagtgattctgctccttcgtgccctcatccaacaaggcttcttgctgctcactacccagctacccctacgtgtggcccgtatcttcatggttcaagatggcagctagagctgctaggtagttaagatctctctcacacactttccttctgtcataattaacacagggttttagctcatgaggccaagcatacacattacttcccactggcacccctatgtaatattaaatgcaaagataccctcaggagtcctgtgctcaaaacaagtacaaaataactttttgttgttgtttgtggtgctggtggttttatttatttattttttctgaaacagggtctcactctgtctcccatgctgaagtgcagtggtgtgatcacagctcatcacaaccttgacctctctgggctcaggggatccactcacttcagcctcccaagtagctgggactacaggaacacgccaccacgctcagctaaattttgtctttttttgtagagatggagtcttgctatgttgcccaggctggtctcaaactcctgggctcaagtgatcagtccacctcagcctcccaaagtactcagattataggtatgagccaccatggcatcaaaataacttggaaagtaggaataattgcttgttgttcctgaaaactgtctcttcgacacttttcagactctgttacatgatcatgacaaaatatacacaaatagacatacagatacacatcagttaaaacctcaagaaatagaaaaataaataaatcataaaatatttaaaaagtggtattctgacacactgcccagaggtacccctgttcagcaattttaaaaaattttaaaaatagccctctccccctccctctcttctccctctccccacggtctccctctgatgccgagccgaagctggactgtactgctgccatctcggctcactgcagcctccctgcctgattctcccgcctcggcctgccgcgtgcctgccattgcgggcgccgccacgcctgactggttttcgtatttttttggtggagacagggtttcactgtgttggccgggctggtctccagctcctgactgcgagtgatctgccagcctcggcctcccgaggtgccgggattgcgggcagagtctcgtccactcagtgctcaatgttgcccaggctggagtgcagtggtgtgatctcagctggctacggcctccgcctcccagccgcctgccttggccccccagggtgccgagattacagcttctgcccggccgccaccccgtctgggatgaagtgaggagcgtctctgcccggccgcccatcgtctgagatgtggggagcgcctctgccccgcccccccgtctgggatgtgaggagcttctctgcccggccaccccgtctgagaagtgaggagcccctccgcccgcagctgccccgtctgagaagtgaggagcccctccgcccgacagccaccctgtctgggaagtgaggagcgtctccgcccagcagccaccccgtctgagaagtgaggagcccctccgcctggcagccgccccgtccgggagggaggcgtgggggtcagcccccgcccggccagccgccccgtcggggagggaggtggggggtcagcccccgcccggccagctatcccgtccgggagggaggtggggggcgcgtccgcctggccgccccatctgggaagtgaggagcccctctgcccagccgccaccccgtctgggaggtgtacccaacagctcattgagaacaggccatgatgacgatggcggttttgtggaatagaaaagggggaaaggtggggaaaagatagagaaatcagattgttgctgtgtctgtgtagaaagaagtagacatgggagacttcattttgttctgtactaagaaaaattcttctgccttaggatgctgttgatctatgaccttacccccaaccctgtgctctctgaaacatgtgctgtgtccactcagggttaaatggattaagggcagtgcaagatgtgctttgttaaacagatgcttgaaggcagcatgctccttaagagtcatcaccactccctaatctcaagtacccagggacacaaacactgcggaaggccgcagggtcctctgcctaggaaaaccagagacctttgttcacttgtttatctgctgaccttccctccactattgtcctgtgaccctgccaaatcaccctctgtgagaaacacccaagaatgatcaattaaaaaaaaaaaatttaaaaataataataggccaggtgcagtggctcacacctgtaatcccagcactttgggaggccgaggctggtgaatcacctgaggtcaggagttcaagaccacgctggccaacatggtggaaaccctgtctccactaaaaatacaaaaattagccgggtgtggtggcaggagcctgtaatcccagctactcgggaggctgaggcaggagaatcgcttgaacccagaaggcagaggttgcaatgagccaagatgatgccactgcactccagcctgggcagcagaatgaaactctgtctcaataataataataataataataataataataataataataataataagcaactctaatgatatttcaaacaatggtccccttttaggtcacactatcaaatcagagaaagatatacttgactagctgtaaaatgcaatttgaggtctaggtgaatgaacaagtaacctctaaatcataaggctattgttacaaactgaatgtttgtattccccccagaattcaaaggggagacagtatccccaaagtgacagtatcagaaggtggggcctttgggaggtaattaggtgatgagggtagagccctcatgaatggaatttgtgcccttaaagatatacttgagagtttgcatcctctttttctgccatgtgagaacatcaaaagactgacatctggtaagatctggaagcatgccttaccagacaccagatatgctaccacttagatgttggatttcccagcctccggaactgtgagaaataactgctgtttaagtcacctggtctatggtaatttggtatagttgcccaaatggactgtgatggttaatactgagtatcaacttgattgaatagaaggatgcaaagtgttcccgggtacatctgtgagggtgctgccaaaggagatttaacatttgagtcagtggactgggaaaggcagaccatcctcaatctgggtgggcaccatctaatcagctgccagcactgccagaataaaagcaggcaaaacatggaaagactagactggtgtagtcttctggcctccatctttctctcatgctgaatgcttcctgccctcaaacattggactccaagttcttcagctttgggacttgaattggcttccttgcttgcagatgacctattgtgggacctaaccctgtgatcatgtgagtcaatactccttaataaactcccctttttatatacatgtatcctattagttctgtccctctagagaaacatgactaatacattgagtaagatagttcctgtcctttttttttttttttaaagagatgggatcttgctatattgcccaggttggtatgcagtggctattcgtaggcacaatcacagcatgctatgaccctgaactcctgggttcaaaagatcctcccacctcagcctcccaagtaactgggaatacaggtacccacacccacacccagctaatttttgtatttttactagggacagcgtttaccatgttggccaggctggtctcgaactcctgacctgaagtgatctgccctccttggcctcccaaagtgctgggattacaggtgtgagccactacgcccagccttttggtttcttatgtgtaggagaggataagtttctttctcagagtgtgctgcagccagacataatatttctccttggcagaaactctgctgttccaatcatacatgtagccattgagttcaatgtgaagatccaggagtgggcgttttctttcttgtctcagtttctgggagaggcactgcaggtacagggatggtgagctgtgagactgctccagcagggacatgtccgcagtacacaggctccagaagaagtcagcttctcggtgaactgtgcacagccctcgcttctgagccttgaattccacattcttcatcgctggcccatccacctccaagaggctgctgtcctccagctggccctctgacaccacatagttctgaataaaaaacatctttggcttccctgctagataagggcatgaatctcccatgaacatcctcctgatgtgatgcagggggagccctgagtgagtctgatccacaccatacacactctgggagcctcctcggctcaccaggacacacacaaagctgtcgtagtctcggtgctcgggcatacaggcaaattggccaagaatctgggatataccatgcatactgagatgcaagaatttctggacttcatagcccagggaagtgaaggtgtctcgaagaagctctgtctcattgccaatgcaatcgattatcaggcagattcctaggggcttgctcttcatcttgtatctctcttcaggtatgctcctgaagttatttgaaggatccttgagactcttttggattgctgcttggagaacattcctgtaacttgtccctgctccttgaacagactgcttgtacttctggatttttgtcttcaggtctattctgtggatgttctttaggcatttttctaataaatccagttgatctggggcaaccagatttagtttctccaactcaaccacaaggtccaagaaactcttctccttgcttatcttgcctcggcccatgtaatccttcatgaggaaaattaatgaggacacatcagatttatccaaatcctcaccaatctctgccatcagcactctatagtccgaaacaaggtgagggttcctgagcaggtgggtctccacagcttttctgtccatcttcaagatacgtttgagcaggtcaaatcgcctcactctgtagagcagttcagccaagtccccgacagacagcttacctctttcccgtaaaatatccagaaggtccctgacattaggtggaaccacatctatagcaacatcccggcacaaaaagagcagcatctccttctcatctgtatcaagtgcttcttcaacctgatggatgacttcagcagacatcctactcttagactagggaagctcacaagggtcttgcagtacagctccgggccagtcaacagaaagccagcaggcagtcaacttcatttctgagggctgacttcatttctttcagaatcctttccagtgggggagttcgtcctgtcgcggccggactctcctgccgctgccacctcagccttcgctcccctagacgccgggaaggcgcacccaagatggaggcaaagaaaccgaaagcctggaagcggacttggtgctgggcgatcgctgttcgcggcgcttctctcctacacctcctcccgtggtccttgttgtctcagctgtcactggacaaaagtccaatagccggcactcactgtgtgaggccgagtccccacccctagctccgggagtcccttttagttgagactcgtcggtgaggctgcaagctcgctgtttcctgctatggcttgtgt

SEQ ID NO: 15266 - RNA, 12883 nt, Homo sapiens
  source 1..12883: mol_type = other RNA
gctgggattacaggcatgagccactgcgcccagccaaacttatctttgtatgtttgttataggcaaaagtaccccaaggttaaggctcagcccaagaggtcaagtgggttcaggaaagaattcaagagcatgctgacagaataaagtgaaagcaagttcattaagaaagtaaaggaataaaagaatggctaccccataggaagagtagccctgatgggctgctgactggctatatttatggttgcttcttgactatacgctaaacaagaggtggcttattcatgagttttccaggaaagaagtggggaggtctggaccttttagaccatacagggtaacttctgaaagttgctatggcagttgtaaactatcatggtgctgtagaagtttcttttagcgtgctaatgtattataattaccatagaatgggcagcaaaggtaaccagaggtctcttctgtcaccatcatggttttggctggtttgggttggcctttctaccacatcctgtcttatcagcagggtcttacagggtcttgtggtcttgggaaaccagtcctgccaaactcctctcattcagtgtaatcactatcaaaattccagaggccctttttacataaatttgcaagtgaatcctaacagttatatgaaaatttagggaaaggtaaacccaatacagccctaacaattttgaaaaagaacaggccagttgcagtggctcacccctcagcactttgggaggtggaggtgggaggattgtttgaggccaggagtttgagaccagcctgggcaacatagcaaggcctcatctctacaaaagaaaaaagaagaacaacaacaacaacaaagttagaggactacatttctggattccaaaacttactacgaagttacaataatcaagacagtgtggtactaccataagatagagcaacagaattgagtccagaaataaacccttatagttagttgatttgtgataagtataaaataattctatagggaaaaaatagtattttcaataagtaatgctaagacaagtgaacatttatgtgcaaaagaatgaggctggatgcttatctcgcactgcatacacaaaaataactcaaaatgggtcaaagagctaaaatcataaaactttagaagaaaacataggggtaacacctcataggcaattgatttagacaatggttttttaggtatgacaccaaaagcataagcaataacataaaaaacagaaatcaagtgaacttcatcaaaatttaaaacttgtactgtatagtatccagaaagtgagaagacaatccatggaatgggagaatatattcacaaagattgtacctgataagaaactagtatccagaatattaaaaagaatgcttacaactcaacaataaaaagacaacccaccgggtgtggtggctcacgcctgtaatcctagcattttgggaggccgaggcaggcagatcacctgagttcaggagttcaagaccagcctggccaacatggcgaaaccctgtctctactaaaaatacaaaaattagccaggcgtgatggtgggtgcctgtaatcccagttactagggaggccgaggcaggagagtcgcttgaactcaggaggtggaggttgcagtgagccgagattgcaccactgcactccaacctgggcgacagagtgagattccatctcagaaaaataaaataaaataacgcagttttaaaatgagaaaggacttgaggccaggcacagtagctaatgtctgtaatgccagcactttgggaagccaaggcagtcagatcacctgaggccaggagttcgagaccagcctggccaacatggtgaaaccctgtctttactaaaaatacaaaaattggctgggcgcggtggctcacgcctgtaatcccagcactttgggaggccaaggcaggcggatcacgaggtcaggagatagagaccatcctggctaacacggtgaaaccctgtctctactaaaaatacaaaaaattagccgggcgtggtggagggcggctgtagtcccagatacttgggaggctgaggcaggagaatggcatgaacccaggaggcggagcttgcagtgagctgagattgcaccactgcactccagcctgggccacagagcgagactccgtctcaaaaaacaatacaaaaattagttgggcatggtggcgagctcctgtaaacccagctactcccaactactagggaggctgaggcaggagaatggcttgaacccagaaggcagaggttacagtgaatcaagataacgccactgcactccaccctgggcgacagagtgagactccgtctcaaaaacaaaaaaataaaaaaaacctcatacactgctggtgggaatataaaatgatgctactactttgaaaagcagtttggcagttcctcaaaaggctaaacatagagttactatatgatgagcactctcacttctaaggtatatgcccagaagaactgaaaacatatatccatataaaaattcatatacgaatattcatagcagcatcatccataatagcaaaaaagtggaaacagtctaaatttcgatcaactgatgaataaactaaatgcggtatatccacacaatagggtattattcagccataaaatgtaatgaagcactggtacactctatagcatagatgaaccttgaaacatgctaagtgaaggaagtcagacacgaaaggccacatgtttatttttataaaatatctagaacaggcaaatcatagagacagaaaatggattattgtttctagaggctgggggaagaggaggattagagtggcagctcactggtatggagtttctaggtagatggaaatgttctggaattagatagtggtgatgattgcacaactctgtaaatatactaaaatccactgcatcatttactttaaaggggcaaattttatggcttgtgaattacatttcaataaaaagaagatgaggaaacctaggatatgtcacaatcccatgccacaaactacttacacttccaatataaaaactatatcaacaatagtttacatcacgttcattgcttgctaaagtaaggtcatgaatgtatcaaaatattttataaaagttaaaatttaggagatccatcatttctcttttcaatccatcactgattcattcaatatatatttatgtgtatgccaggctcttcatcaggtaaagtgtttaggagagatataaagataaaactgatgagaattctgcacttgagctacagcatactttccaagaattacagcatgagatataaaatgaaaagaaggcttggaggagattcacacgaaatagtactgttcaggagagggggcgataattccaatggaagagataactgacttcatggaggatagaaggagatggtatttgaactgcccttgaagtatggttatattttggggatgtggagatgtggggtagggtgatatgctggggttccagatggtccagaaatatacaatcaccagaaccaaagatccagaggtaggagatatgagctgttcaatttggctgagctaacagtgtttggagtgggatcttgaagaagctgaaaatgaagataccaactagacagtcagagaaagacttccaatgtttgactgaactgcaattttattgtgtatgcattgaagaatctttttttttttttttgtattctctaaagatttttaaaatattttaagttctggatacaagtgcaggatgtgcgggtttgttacataggtaaacgtgtcccatggtggtttgctgcacctatcaacctatcacctaggtattaagccccacatgcattagctagttatcctgatgctctccccgctacggcccctgcatcaggccccagtgtgtgttgatctcatccctgtgtccgtgtgttctcattgttcagcttccgcttacaagtgagaacatgtggtgtttggtttcctgctcctctgttagtttgctgaggataatggcttccagcttcatccatgtccctgcaaaggacatgatctcattccttttttaaaaaaaaaaacaaaattatttccataggtgtttggggaacaggtggtatctggttacatgcgtaagtaattaagtggttacttgtgagattctggtgcacccatcacctgagcagtatacactgaacccaatttgtattcttttatccttcacccccctcccaccctttcccctaagtccccaaagtccattgtatccttcttatgcctttgcatcctcatagcttatctcccacttatgagtgagaacatacaatgtttggttttccattcctcagttacttcctttagagtaatagtctccaggttgctgtgaatgtcattaattcattcctttttatggctgagtagtgtttaggtgaggttatttgtaagtaattaatattgagtaaataagattcatccatagtggcaaagccacataacttctaagtatcttaaactatatctaaatggtaccaaaacatgcagtcaattctaaaagctcagctaatgatatttcataatataggaaaatattcacaacatatttttgtgtaaaaaaaagcagacttcaaaatggaatatgcattatgattccaatcatgtaaaagctatacatgaacacatacaaagattaacagatataaacaaatggaagaatgaatggagagatagatgatagacagattgagtggtggtggagaataacagatttaaaaagaaattgtgcctttctatattttcaaaaccatttaaataagtattacctttggagttagaaaatgatatgtattttaaatccataattcaactacttatctatatgatgtcaaactggattaggctgaattatcagcaagtgaataaaacagttccttcatccatggagaaacatccatttatgacattcttggaattcctcttgttagaattctttatgaatttaaaatagaaacatggccagactcaagatttcaatacaaacattactttttcacgttcagtaataaccaattaaaagaattaatgaaaaatctgattcactgtatcaccaaaagctgtaatggctgcactgcacagtattccatggtgtatatgtaccacattttctttatccagtctatctttgatgggcatttgctattgtgtctttgctattgtgaagagtgctgcaatgaacaaaaatgtgcatgtatctttataataaaatggtttatattcctttgggtatatacccagtaatgggattgctgggacaaatagtatttctagttctagatctttgaggaatagccacacacacttccacaacggttgaactaatttacattcccaccaacaatgtaaaagtgttcctacttctccacagcctcgccagcatctgttgttttttgactttttaataatcaccattctgaccggcatgagatggtatctcattgtggttctcctttgcatttctctaatgatcagtaaggttgagcttttttttatatgtttgttggccacataaatgtcttcttttgagaagtgtctgttcatgtcctttgtccactttttgatggggttgtttttttccttgtaaatttgttttaagttccttgtaggttctggatattagacctttgtcagatggatagattgcaaaaatgttctcccattctgtaggttgcctgttcactctaatgatagtttcttttgctgtgcaggagctctttagtttaattagatcccatttgtaatttttgcttttgttgcaattgcttttgatgtttttgtcatgaaacctttgcttgtgcctatgtcttgaatggtattaaatagattttcttctagggtttttatagttttaggttttacattaagtctttaatcttgagttaatttttgtataaggtgtaaggaaggggtcagtttcaattttctgcatatggctagccagttttcccagcaccatttattaaatagggaatcttttccccattgcttgtttttgtcaggtttgtcgatgatcagatggctgtagatgtgtggtcttctttctctggtctctattctgttccattggtctatgtgtctgtttttgtaccagtaccatgccattttggctactgtagccttgcagtatactttgaagttgggtagtgtgatgcttccagctttgttctttttgcttattgttgtcttggttatacgggctcttttttggttccatttgaattttaaagtagtttttttctaattctgtgaagaatgtcaatagtagtttaatgggaatagcaatgaacctataaattactttgggtagtatggccattttcatgatattgattcttcctatccacgagaatggaatgttttttcatttgtgtcctctcttatttccttgagcagtggtttgtagttctccttgaagagatccttcacatcttattagctgtattcctaggtattttattctctttctagcaactgtgaatgggagttcattcatgatttggctctctgcttgtgtattgttggtgtatagaatgcttgtgatttctgcacattgattttgtatcctgagactttgctgaagttgcttatcagcttaaggaacttttgggtggagataatggggttttctagatatagtatcatgtcatctgcaaacacagttttacttcctcttttcctatttgaataccccttatttgtttctcttgcctgattttcttggccagaacttccaatactatgttaaataggagtggtgagacggcatccctgtcttgtgccagttttcaaggggaatgcttccagcttttgcccattcagtatgataatggctgtgggtttgtcataaatggttattattttgagatattttccatcaatacctagtttattgagagtttttaacatgaagcaacgttgaattttattgaaggccttttctgtatctattgagataatcatgtggtttttgtctttagttctgtttatgtgatgaattatgtttcttgatttgcgtatgttgaaccagccttgcatcccagggatgaagccaacattccaaacattttatttattatttatttatttatttatttttgagacagagtctcgcactgtcgcccaggctggagtgcagtggcaagatctcagctcgctgcaagctccacctcccaggttcatgccgttctcttgcctcggcctcccaaatagcagggactacaggcgaccgccacaacgcctggctaattttttgtatttttagtagagacggggttttacatgttagccaggatggtcttgatctcctgacctcgtgatccgcccgccttggcctcccaaagggctgggattataggcgtgagccaccgcacccggcctccaaacattttaatctcataacaatgcatcacttgggttaactaggttgagataaatataaactgtcaattttttttcccctcacataaaagtccagaggtaggtaattagggctgacacagtgattccagtgattctgctccttcgtgccctcatccaacaaggcttcttgctgctcactacccagctacccctacgtgtggcccgtatcttcatggttcaagatggcagctagagctgctaggtagttaagatctctctcacacactttccttctgtcataattaacacagggttttagctcatgaggccaagcatacacattacttcccactggcacccctatgtaatattaaatgcaaagataccctcaggagtcctgtgctcaaaacaagtacaaaataactttttgttgttgtttgtggtgctggtggttttatttatttattttttctgaaacagggtctcactctgtctcccatgctgaagtgcagtggtgtgatcacagctcatcacaaccttgacctctctgggctcaggggatccactcacttcagcctcccaagtagctgggactacaggaacacgccaccacgctcagctaaattttgtctttttttgtagagatggagtcttgctatgttgcccaggctggtctcaaactcctgggctcaagtgatcagtccacctcagcctcccaaagtactcagattataggtatgagccaccatggcatcaaaataacttggaaagtaggaataattgcttgttgttcctgaaaactgtctcttcgacacttttcagactctgttacatgatcatgacaaaatatacacaaatagacatacagatacacatcagttaaaacctcaagaaatagaaaaataaataaatcataaaatatttaaaaagtggtattctgacacactgcccagaggtacccctgttcagcaattttaaaaaattttaaaaatagccctctccccctccctctcttctccctctccccacggtctccctctgatgccgagccgaagctggactgtactgctgccatctcggctcactgcagcctccctgcctgattctcccgcctcggcctgccgcgtgcctgccattgcgggcgccgccacgcctgactggttttcgtatttttttggtggagacagggtttcactgtgttggccgggctggtctccagctcctgactgcgagtgatctgccagcctcggcctcccgaggtgccgggattgcgggcagagtctcgtccactcagtgctcaatgttgcccaggctggagtgcagtggtgtgatctcagctggctacggcctccgcctcccagccgcctgccttggccccccagggtgccgagattacagcttctgcccggccgccaccccgtctgggatgaagtgaggagcgtctctgcccggccgcccatcgtctgagatgtggggagcgcctctgccccgcccccccgtctgggatgtgaggagcttctctgcccggccaccccgtctgagaagtgaggagcccctccgcccgcagctgccccgtctgagaagtgaggagcccctccgcccgacagccaccctgtctgggaagtgaggagcgtctccgcccagcagccaccccgtctgagaagtgaggagcccctccgcctggcagccgccccgtccgggagggaggcgtgggggtcagcccccgcccggccagccgccccgtcggggagggaggtggggggtcagcccccgcccggccagctatcccgtccgggagggaggtggggggcgcgtccgcctggccgccccatctgggaagtgaggagcccctctgcccagccgccaccccgtctgggaggtgtacccaacagctcattgagaacaggccatgatgacgatggcggttttgtggaatagaaaagggggaaaggtggggaaaagatagagaaatcagattgttgctgtgtctgtgtagaaagaagtagacatgggagacttcattttgttctgtactaagaaaaattcttctgccttaggatgctgttgatctatgaccttacccccaaccctgtgctctctgaaacatgtgctgtgtccactcagggttaaatggattaagggcagtgcaagatgtgctttgttaaacagatgcttgaaggcagcatgctccttaagagtcatcaccactccctaatctcaagtacccagggacacaaacactgcggaaggccgcagggtcctctgcctaggaaaaccagagacctttgttcacttgtttatctgctgaccttccctccactattgtcctgtgaccctgccaaatcaccctctgtgagaaacacccaagaatgatcaattaaaaaaaaaaaatttaaaaataataataggccaggtgcagtggctcacacctgtaatcccagcactttgggaggccgaggctggtgaatcacctgaggtcaggagttcaagaccacgctggccaacatggtggaaaccctgtctccactaaaaatacaaaaattagccgggtgtggtggcaggagcctgtaatcccagctactcgggaggctgaggcaggagaatcgcttgaacccagaaggcagaggttgcaatgagccaagatgatgccactgcactccagcctgggcagcagaatgaaactctgtctcaataataataataataataataataataataataataataataataagcaactctaatgatatttcaaacaatggtccccttttaggtcacactatcaaatcagagaaagatatacttgactagctgtaaaatgcaatttgaggtctaggtgaatgaacaagtaacctctaaatcataaggctattgttacaaactgaatgtttgtattccccccagaattcaaaggggagacagtatccccaaagtgacagtatcagaaggtggggcctttgggaggtaattaggtgatgagggtagagccctcatgaatggaatttgtgcccttaaagatatacttgagagtttgcatcctctttttctgccatgtgagaacatcaaaagactgacatctggtaagatctggaagcatgccttaccagacaccagatatgctaccacttagatgttggatttcccagcctccggaactgtgagaaataactgctgtttaagtcacctggtctatggtaatttggtatagttgcccaaatggactgtgatggttaatactgagtatcaacttgattgaatagaaggatgcaaagtgttcccgggtacatctgtgagggtgctgccaaaggagatttaacatttgagtcagtggactgggaaaggcagaccatcctcaatctgggtgggcaccatctaatcagctgccagcactgccagaataaaagcaggcaaaacatggaaagactagactggtgtagtcttctggcctccatctttctctcatgctgaatgcttcctgccctcaaacattggactccaagttcttcagctttgggacttgaattggcttccttgcttgcagatgacctattgtgggacctaaccctgtgatcatgtgagtcaatactccttaataaactcccctttttatatacatgtatcctattagttctgtccctctagagaaacatgactaatacattgagtaagatagttcctgtcctttttttttttttttaaagagatgggatcttgctatattgcccaggttggtatgcagtggctattcgtaggcacaatcacagcatgctatgaccctgaactcctgggttcaaaagatcctcccacctcagcctcccaagtaactgggaatacaggtacccacacccacacccagctaatttttgtatttttactagggacagcgtttaccatgttggccaggctggtctcgaactcctgacctgaagtgatctgccctccttggcctcccaaagtgctgggattacaggtgtgagccactacgcccagccttttggtttcttatgtgtaggagaggataagtttctttctcagagtgtgctgcagccagacataatatttctccttggcagaaactctgctgttccaatcatacatgtagccattgagttcaatgtgaagatccaggagtgggcgttttctttcttgtctcagtttctgggagaggcactgcaggtacagggatggtgagctgtgagactgctccagcagggacatgtccgcagtacacaggctccagaagaagtcagcttctcggtgaactgtgcacagccctcgcttctgagccttgaattccacattcttcatcgctggcccatccacctccaagaggctgctgtcctccagctggccctctgacaccacatagttctgaataaaaaacatctttggcttccctgctagataagggcatgaatctcccatgaacatcctcctgatgtgatgcagggggagccctgagtgagtctgatccacaccatacacactctgggagcctcctcggctcaccaggacacacacaaagctgtcgtagtctcggtgctcgggcatacaggcaaattggccaagaatctgggatataccatgcatactgagatgcaagaatttctggacttcatagcccagggaagtgaaggtgtctcgaagaagctctgtctcattgccaatgcaatcgattatcaggcagattcctaggggcttgctcttcatcttgtatctctcttcaggtatgctctgaggcaaaaaagcttctgattcctgaatggatttcttcactggttcttgttgagcgccaagctgttccttaagtctttgttctttacttctcccattatggagcctgaagttatttgaaggatccttgagactcttttggattgctgcttggagaacattcctgtaacttgtccctgctccttgaacagactgcttgtacttctggatttttgtcttcaggtctattctgtggatgttctttaggcatttttctaataaatccagttgatctggggcaaccagatttagtttctccaactcaaccacaaggtccaagaaactcttctccttgcttatcttgcctcggcccatgtaatccttcatgaggaaaattaatgaggacacatcagatttatccaaatcctcaccaatctctgccatcagcactcgtcctgtcgcggccggactctcctgccgctgccacctcagccttcgctcccctagacgccgggaaggcgcacccaagatggaggcaaagaaaccgaaagcctggaagcggacttggtgctgggcgatcgctgttcgcggcgcttctctcctacacctcctcccgtggtccttgttgtctcagctgtcactggacaaaagtccaatagccggcactcactgtgtgaggccgagtccccacccctagctccgggagtcccttttagttgagactcgtcggtgaggctgcaagctcgctgtttcctgctatggcttgtgt

SEQ ID NO: 15267 - RNA, 13301 nt, Homo sapiens
  source 1..13301: mol_type = other RNA
gctgggattacaggcatgagccactgcgcccagccaaacttatctttgtatgtttgttataggcaaaagtaccccaaggttaaggctcagcccaagaggtcaagtgggttcaggaaagaattcaagagcatgctgacagaataaagtgaaagcaagttcattaagaaagtaaaggaataaaagaatggctaccccataggaagagtagccctgatgggctgctgactggctatatttatggttgcttcttgactatacgctaaacaagaggtggcttattcatgagttttccaggaaagaagtggggaggtctggaccttttagaccatacagggtaacttctgaaagttgctatggcagttgtaaactatcatggtgctgtagaagtttcttttagcgtgctaatgtattataattaccatagaatgggcagcaaaggtaaccagaggtctcttctgtcaccatcatggttttggctggtttgggttggcctttctaccacatcctgtcttatcagcagggtcttacagggtcttgtggtcttgggaaaccagtcctgccaaactcctctcattcagtgtaatcactatcaaaattccagaggccctttttacataaatttgcaagtgaatcctaacagttatatgaaaatttagggaaaggtaaacccaatacagccctaacaattttgaaaaagaacaggccagttgcagtggctcacccctcagcactttgggaggtggaggtgggaggattgtttgaggccaggagtttgagaccagcctgggcaacatagcaaggcctcatctctacaaaagaaaaaagaagaacaacaacaacaacaaagttagaggactacatttctggattccaaaacttactacgaagttacaataatcaagacagtgtggtactaccataagatagagcaacagaattgagtccagaaataaacccttatagttagttgatttgtgataagtataaaataattctatagggaaaaaatagtattttcaataagtaatgctaagacaagtgaacatttatgtgcaaaagaatgaggctggatgcttatctcgcactgcatacacaaaaataactcaaaatgggtcaaagagctaaaatcataaaactttagaagaaaacataggggtaacacctcataggcaattgatttagacaatggttttttaggtatgacaccaaaagcataagcaataacataaaaaacagaaatcaagtgaacttcatcaaaatttaaaacttgtactgtatagtatccagaaagtgagaagacaatccatggaatgggagaatatattcacaaagattgtacctgataagaaactagtatccagaatattaaaaagaatgcttacaactcaacaataaaaagacaacccaccgggtgtggtggctcacgcctgtaatcctagcattttgggaggccgaggcaggcagatcacctgagttcaggagttcaagaccagcctggccaacatggcgaaaccctgtctctactaaaaatacaaaaattagccaggcgtgatggtgggtgcctgtaatcccagttactagggaggccgaggcaggagagtcgcttgaactcaggaggtggaggttgcagtgagccgagattgcaccactgcactccaacctgggcgacagagtgagattccatctcagaaaaataaaataaaataacgcagttttaaaatgagaaaggacttgaggccaggcacagtagctaatgtctgtaatgccagcactttgggaagccaaggcagtcagatcacctgaggccaggagttcgagaccagcctggccaacatggtgaaaccctgtctttactaaaaatacaaaaattggctgggcgcggtggctcacgcctgtaatcccagcactttgggaggccaaggcaggcggatcacgaggtcaggagatagagaccatcctggctaacacggtgaaaccctgtctctactaaaaatacaaaaaattagccgggcgtggtggagggcggctgtagtcccagatacttgggaggctgaggcaggagaatggcatgaacccaggaggcggagcttgcagtgagctgagattgcaccactgcactccagcctgggccacagagcgagactccgtctcaaaaaacaatacaaaaattagttgggcatggtggcgagctcctgtaaacccagctactcccaactactagggaggctgaggcaggagaatggcttgaacccagaaggcagaggttacagtgaatcaagataacgccactgcactccaccctgggcgacagagtgagactccgtctcaaaaacaaaaaaataaaaaaaacctcatacactgctggtgggaatataaaatgatgctactactttgaaaagcagtttggcagttcctcaaaaggctaaacatagagttactatatgatgagcactctcacttctaaggtatatgcccagaagaactgaaaacatatatccatataaaaattcatatacgaatattcatagcagcatcatccataatagcaaaaaagtggaaacagtctaaatttcgatcaactgatgaataaactaaatgcggtatatccacacaatagggtattattcagccataaaatgtaatgaagcactggtacactctatagcatagatgaaccttgaaacatgctaagtgaaggaagtcagacacgaaaggccacatgtttatttttataaaatatctagaacaggcaaatcatagagacagaaaatggattattgtttctagaggctgggggaagaggaggattagagtggcagctcactggtatggagtttctaggtagatggaaatgttctggaattagatagtggtgatgattgcacaactctgtaaatatactaaaatccactgcatcatttactttaaaggggcaaattttatggcttgtgaattacatttcaataaaaagaagatgaggaaacctaggatatgtcacaatcccatgccacaaactacttacacttccaatataaaaactatatcaacaatagtttacatcacgttcattgcttgctaaagtaaggtcatgaatgtatcaaaatattttataaaagttaaaatttaggagatccatcatttctcttttcaatccatcactgattcattcaatatatatttatgtgtatgccaggctcttcatcaggtaaagtgtttaggagagatataaagataaaactgatgagaattctgcacttgagctacagcatactttccaagaattacagcatgagatataaaatgaaaagaaggcttggaggagattcacacgaaatagtactgttcaggagagggggcgataattccaatggaagagataactgacttcatggaggatagaaggagatggtatttgaactgcccttgaagtatggttatattttggggatgtggagatgtggggtagggtgatatgctggggttccagatggtccagaaatatacaatcaccagaaccaaagatccagaggtaggagatatgagctgttcaatttggctgagctaacagtgtttggagtgggatcttgaagaagctgaaaatgaagataccaactagacagtcagagaaagacttccaatgtttgactgaactgcaattttattgtgtatgcattgaagaatctttttttttttttttgtattctctaaagatttttaaaatattttaagttctggatacaagtgcaggatgtgcgggtttgttacataggtaaacgtgtcccatggtggtttgctgcacctatcaacctatcacctaggtattaagccccacatgcattagctagttatcctgatgctctccccgctacggcccctgcatcaggccccagtgtgtgttgatctcatccctgtgtccgtgtgttctcattgttcagcttccgcttacaagtgagaacatgtggtgtttggtttcctgctcctctgttagtttgctgaggataatggcttccagcttcatccatgtccctgcaaaggacatgatctcattccttttttaaaaaaaaaaacaaaattatttccataggtgtttggggaacaggtggtatctggttacatgcgtaagtaattaagtggttacttgtgagattctggtgcacccatcacctgagcagtatacactgaacccaatttgtattcttttatccttcacccccctcccaccctttcccctaagtccccaaagtccattgtatccttcttatgcctttgcatcctcatagcttatctcccacttatgagtgagaacatacaatgtttggttttccattcctcagttacttcctttagagtaatagtctccaggttgctgtgaatgtcattaattcattcctttttatggctgagtagtgtttaggtgaggttatttgtaagtaattaatattgagtaaataagattcatccatagtggcaaagccacataacttctaagtatcttaaactatatctaaatggtaccaaaacatgcagtcaattctaaaagctcagctaatgatatttcataatataggaaaatattcacaacatatttttgtgtaaaaaaaagcagacttcaaaatggaatatgcattatgattccaatcatgtaaaagctatacatgaacacatacaaagattaacagatataaacaaatggaagaatgaatggagagatagatgatagacagattgagtggtggtggagaataacagatttaaaaagaaattgtgcctttctatattttcaaaaccatttaaataagtattacctttggagttagaaaatgatatgtattttaaatccataattcaactacttatctatatgatgtcaaactggattaggctgaattatcagcaagtgaataaaacagttccttcatccatggagaaacatccatttatgacattcttggaattcctcttgttagaattctttatgaatttaaaatagaaacatggccagactcaagatttcaatacaaacattactttttcacgttcagtaataaccaattaaaagaattaatgaaaaatctgattcactgtatcaccaaaagctgtaatggctgcactgcacagtattccatggtgtatatgtaccacattttctttatccagtctatctttgatgggcatttgctattgtgtctttgctattgtgaagagtgctgcaatgaacaaaaatgtgcatgtatctttataataaaatggtttatattcctttgggtatatacccagtaatgggattgctgggacaaatagtatttctagttctagatctttgaggaatagccacacacacttccacaacggttgaactaatttacattcccaccaacaatgtaaaagtgttcctacttctccacagcctcgccagcatctgttgttttttgactttttaataatcaccattctgaccggcatgagatggtatctcattgtggttctcctttgcatttctctaatgatcagtaaggttgagcttttttttatatgtttgttggccacataaatgtcttcttttgagaagtgtctgttcatgtcctttgtccactttttgatggggttgtttttttccttgtaaatttgttttaagttccttgtaggttctggatattagacctttgtcagatggatagattgcaaaaatgttctcccattctgtaggttgcctgttcactctaatgatagtttcttttgctgtgcaggagctctttagtttaattagatcccatttgtaatttttgcttttgttgcaattgcttttgatgtttttgtcatgaaacctttgcttgtgcctatgtcttgaatggtattaaatagattttcttctagggtttttatagttttaggttttacattaagtctttaatcttgagttaatttttgtataaggtgtaaggaaggggtcagtttcaattttctgcatatggctagccagttttcccagcaccatttattaaatagggaatcttttccccattgcttgtttttgtcaggtttgtcgatgatcagatggctgtagatgtgtggtcttctttctctggtctctattctgttccattggtctatgtgtctgtttttgtaccagtaccatgccattttggctactgtagccttgcagtatactttgaagttgggtagtgtgatgcttccagctttgttctttttgcttattgttgtcttggttatacgggctcttttttggttccatttgaattttaaagtagtttttttctaattctgtgaagaatgtcaatagtagtttaatgggaatagcaatgaacctataaattactttgggtagtatggccattttcatgatattgattcttcctatccacgagaatggaatgttttttcatttgtgtcctctcttatttccttgagcagtggtttgtagttctccttgaagagatccttcacatcttattagctgtattcctaggtattttattctctttctagcaactgtgaatgggagttcattcatgatttggctctctgcttgtgtattgttggtgtatagaatgcttgtgatttctgcacattgattttgtatcctgagactttgctgaagttgcttatcagcttaaggaacttttgggtggagataatggggttttctagatatagtatcatgtcatctgcaaacacagttttacttcctcttttcctatttgaataccccttatttgtttctcttgcctgattttcttggccagaacttccaatactatgttaaataggagtggtgagacggcatccctgtcttgtgccagttttcaaggggaatgcttccagcttttgcccattcagtatgataatggctgtgggtttgtcataaatggttattattttgagatattttccatcaatacctagtttattgagagtttttaacatgaagcaacgttgaattttattgaaggccttttctgtatctattgagataatcatgtggtttttgtctttagttctgtttatgtgatgaattatgtttcttgatttgcgtatgttgaaccagccttgcatcccagggatgaagccaacattccaaacattttatttattatttatttatttatttatttttgagacagagtctcgcactgtcgcccaggctggagtgcagtggcaagatctcagctcgctgcaagctccacctcccaggttcatgccgttctcttgcctcggcctcccaaatagcagggactacaggcgaccgccacaacgcctggctaattttttgtatttttagtagagacggggttttacatgttagccaggatggtcttgatctcctgacctcgtgatccgcccgccttggcctcccaaagggctgggattataggcgtgagccaccgcacccggcctccaaacattttaatctcataacaatgcatcacttgggttaactaggttgagataaatataaactgtcaattttttttcccctcacataaaagtccagaggtaggtaattagggctgacacagtgattccagtgattctgctccttcgtgccctcatccaacaaggcttcttgctgctcactacccagctacccctacgtgtggcccgtatcttcatggttcaagatggcagctagagctgctaggtagttaagatctctctcacacactttccttctgtcataattaacacagggttttagctcatgaggccaagcatacacattacttcccactggcacccctatgtaatattaaatgcaaagataccctcaggagtcctgtgctcaaaacaagtacaaaataactttttgttgttgtttgtggtgctggtggttttatttatttattttttctgaaacagggtctcactctgtctcccatgctgaagtgcagtggtgtgatcacagctcatcacaaccttgacctctctgggctcaggggatccactcacttcagcctcccaagtagctgggactacaggaacacgccaccacgctcagctaaattttgtctttttttgtagagatggagtcttgctatgttgcccaggctggtctcaaactcctgggctcaagtgatcagtccacctcagcctcccaaagtactcagattataggtatgagccaccatggcatcaaaataacttggaaagtaggaataattgcttgttgttcctgaaaactgtctcttcgacacttttcagactctgttacatgatcatgacaaaatatacacaaatagacatacagatacacatcagttaaaacctcaagaaatagaaaaataaataaatcataaaatatttaaaaagtggtattctgacacactgcccagaggtacccctgttcagcaattttaaaaaattttaaaaatagccctctccccctccctctcttctccctctccccacggtctccctctgatgccgagccgaagctggactgtactgctgccatctcggctcactgcagcctccctgcctgattctcccgcctcggcctgccgcgtgcctgccattgcgggcgccgccacgcctgactggttttcgtatttttttggtggagacagggtttcactgtgttggccgggctggtctccagctcctgactgcgagtgatctgccagcctcggcctcccgaggtgccgggattgcgggcagagtctcgtccactcagtgctcaatgttgcccaggctggagtgcagtggtgtgatctcagctggctacggcctccgcctcccagccgcctgccttggccccccagggtgccgagattacagcttctgcccggccgccaccccgtctgggatgaagtgaggagcgtctctgcccggccgcccatcgtctgagatgtggggagcgcctctgccccgcccccccgtctgggatgtgaggagcttctctgcccggccaccccgtctgagaagtgaggagcccctccgcccgcagctgccccgtctgagaagtgaggagcccctccgcccgacagccaccctgtctgggaagtgaggagcgtctccgcccagcagccaccccgtctgagaagtgaggagcccctccgcctggcagccgccccgtccgggagggaggcgtgggggtcagcccccgcccggccagccgccccgtcggggagggaggtggggggtcagcccccgcccggccagctatcccgtccgggagggaggtggggggcgcgtccgcctggccgccccatctgggaagtgaggagcccctctgcccagccgccaccccgtctgggaggtgtacccaacagctcattgagaacaggccatgatgacgatggcggttttgtggaatagaaaagggggaaaggtggggaaaagatagagaaatcagattgttgctgtgtctgtgtagaaagaagtagacatgggagacttcattttgttctgtactaagaaaaattcttctgccttaggatgctgttgatctatgaccttacccccaaccctgtgctctctgaaacatgtgctgtgtccactcagggttaaatggattaagggcagtgcaagatgtgctttgttaaacagatgcttgaaggcagcatgctccttaagagtcatcaccactccctaatctcaagtacccagggacacaaacactgcggaaggccgcagggtcctctgcctaggaaaaccagagacctttgttcacttgtttatctgctgaccttccctccactattgtcctgtgaccctgccaaatcaccctctgtgagaaacacccaagaatgatcaattaaaaaaaaaaaatttaaaaataataataggccaggtgcagtggctcacacctgtaatcccagcactttgggaggccgaggctggtgaatcacctgaggtcaggagttcaagaccacgctggccaacatggtggaaaccctgtctccactaaaaatacaaaaattagccgggtgtggtggcaggagcctgtaatcccagctactcgggaggctgaggcaggagaatcgcttgaacccagaaggcagaggttgcaatgagccaagatgatgccactgcactccagcctgggcagcagaatgaaactctgtctcaataataataataataataataataataataataataataataataagcaactctaatgatatttcaaacaatggtccccttttaggtcacactatcaaatcagagaaagatatacttgactagctgtaaaatgcaatttgaggtctaggtgaatgaacaagtaacctctaaatcataaggctattgttacaaactgaatgtttgtattccccccagaattcaaaggggagacagtatccccaaagtgacagtatcagaaggtggggcctttgggaggtaattaggtgatgagggtagagccctcatgaatggaatttgtgcccttaaagatatacttgagagtttgcatcctctttttctgccatgtgagaacatcaaaagactgacatctggtaagatctggaagcatgccttaccagacaccagatatgctaccacttagatgttggatttcccagcctccggaactgtgagaaataactgctgtttaagtcacctggtctatggtaatttggtatagttgcccaaatggactgtgatggttaatactgagtatcaacttgattgaatagaaggatgcaaagtgttcccgggtacatctgtgagggtgctgccaaaggagatttaacatttgagtcagtggactgggaaaggcagaccatcctcaatctgggtgggcaccatctaatcagctgccagcactgccagaataaaagcaggcaaaacatggaaagactagactggtgtagtcttctggcctccatctttctctcatgctgaatgcttcctgccctcaaacattggactccaagttcttcagctttgggacttgaattggcttccttgcttgcagatgacctattgtgggacctaaccctgtgatcatgtgagtcaatactccttaataaactcccctttttatatacatgtatcctattagttctgtccctctagagaaacatgactaatacattgagtaagatagttcctgtcctttttttttttttttaaagagatgggatcttgctatattgcccaggttggtatgcagtggctattcgtaggcacaatcacagcatgctatgaccctgaactcctgggttcaaaagatcctcccacctcagcctcccaagtaactgggaatacaggtacccacacccacacccagctaatttttgtatttttactagggacagcgtttaccatgttggccaggctggtctcgaactcctgacctgaagtgatctgccctccttggcctcccaaagtgctgggattacaggtgtgagccactacgcccagccttttggtttcttatgtgtaggagaggataagtttctttctcagagtgtgctgcagccagacataatatttctccttggcagaaactctgctgttccaatcatacatgtagccattgagttcaatgtgaagatccaggagtgggcgttttctttcttgtctcagtttctgggagaggcactgcaggtacagggatggtgagctgtgagactgctccagcagggacatgtccgcagtacacaggctccagaagaagtcagcttctcggtgaactgtgcacagccctcgcttctgagccttgaattccacattcttcatcgctggcccatccacctccaagaggctgctgtcctccagctggccctctgacaccacatagttctgaataaaaaacatctttggcttccctgctagataagggcatgaatctcccatgaacatcctcctgatgtgatgcagggggagccctgagtgagtctgatccacaccatacacactctgggagcctcctcggctcaccaggacacacacaaagctgtcgtagtctcggtgctcgggcatacaggcaaattggccaagaatctgggatataccatgcatactgagatgcaagaatttctggacttcatagcccagggaagtgaaggtgtctcgaagaagctctgtctcattgccaatgcaatcgattatcaggcagattcctaggggcttgctcttcatcttgtatctctcttcaggtatgctctgaggcaaaaaagcttctgattcctgaatggatttcttcactggttcttgttgagcgccaagctgttccttaagtctttgttctttacttctcccattatggagcctgaagttatttgaaggatccttgagactcttttggattgctgcttggagaacattcctgtaacttgtccctgctccttgaacagactgcttgtacttctggatttttgtcttcaggtctattctgtggatgttctttaggcatttttctaataaatccagttgatctggggcaaccagatttagtttctccaactcaaccacaaggtccaagaaactcttctccttgcttatcttgcctcggcccatgtaatccttcatgaggaaaattaatgaggacacatcagatttatccaaatcctcaccaatctctgccatcagcactctatagtccgaaacaaggtgagggttcctgagcaggtgggtctccacagcttttctgtccatcttcaagatacgtttgagcaggtcaaatcgcctcactctgtagagcagttcagccaagtccccgacagacagcttacctctttcccgtaaaatatccagaaggtccctgacattaggtggaaccacatctatagcaacatcccggcacaaaaagagcagcatctccttctcatctgtatcaagtgcttcttcaacctgatggatgacttcagcagacatcctactcttagactagggaagctcacaagggtcttgcagtacagctccgggccagtcaacagaaagccagcaggcagtcaacttcatttctgagggctgacttcatttctttcagaatcctttccagtgggggagttcgtcctgtcgcggccggactctcctgccgctgccacctcagccttcgctcccctagacgccgggaaggcgcacccaagatggaggcaaagaaaccgaaagcctggaagcggacttggtgctgggcgatcgctgttcgcggcgcttctctcctacacctcctcccgtggtccttgttgtctcagctgtcactggacaaaagtccaatagccggcactcactgtgtgaggccgagtccccacccctagctccgggagtcccttttagttgagactcgtcggtgaggctgcaagctcgctgtttcctgctatggcttgtgt

SEQ ID NO: 15268 - RNA, 13169 nt, Homo sapiens
  source 1..13169: mol_type = other RNA
gctgggattacaggcatgagccactgcgcccagccaaacttatctttgtatgtttgttataggcaaaagtaccccaaggttaaggctcagcccaagaggtcaagtgggttcaggaaagaattcaagagcatgctgacagaataaagtgaaagcaagttcattaagaaagtaaaggaataaaagaatggctaccccataggaagagtagccctgatgggctgctgactggctatatttatggttgcttcttgactatacgctaaacaagaggtggcttattcatgagttttccaggaaagaagtggggaggtctggaccttttagaccatacagggtaacttctgaaagttgctatggcagttgtaaactatcatggtgctgtagaagtttcttttagcgtgctaatgtattataattaccatagaatgggcagcaaaggtaaccagaggtctcttctgtcaccatcatggttttggctggtttgggttggcctttctaccacatcctgtcttatcagcagggtcttacagggtcttgtggtcttgggaaaccagtcctgccaaactcctctcattcagtgtaatcactatcaaaattccagaggccctttttacataaatttgcaagtgaatcctaacagttatatgaaaatttagggaaaggtaaacccaatacagccctaacaattttgaaaaagaacaggccagttgcagtggctcacccctcagcactttgggaggtggaggtgggaggattgtttgaggccaggagtttgagaccagcctgggcaacatagcaaggcctcatctctacaaaagaaaaaagaagaacaacaacaacaacaaagttagaggactacatttctggattccaaaacttactacgaagttacaataatcaagacagtgtggtactaccataagatagagcaacagaattgagtccagaaataaacccttatagttagttgatttgtgataagtataaaataattctatagggaaaaaatagtattttcaataagtaatgctaagacaagtgaacatttatgtgcaaaagaatgaggctggatgcttatctcgcactgcatacacaaaaataactcaaaatgggtcaaagagctaaaatcataaaactttagaagaaaacataggggtaacacctcataggcaattgatttagacaatggttttttaggtatgacaccaaaagcataagcaataacataaaaaacagaaatcaagtgaacttcatcaaaatttaaaacttgtactgtatagtatccagaaagtgagaagacaatccatggaatgggagaatatattcacaaagattgtacctgataagaaactagtatccagaatattaaaaagaatgcttacaactcaacaataaaaagacaacccaccgggtgtggtggctcacgcctgtaatcctagcattttgggaggccgaggcaggcagatcacctgagttcaggagttcaagaccagcctggccaacatggcgaaaccctgtctctactaaaaatacaaaaattagccaggcgtgatggtgggtgcctgtaatcccagttactagggaggccgaggcaggagagtcgcttgaactcaggaggtggaggttgcagtgagccgagattgcaccactgcactccaacctgggcgacagagtgagattccatctcagaaaaataaaataaaataacgcagttttaaaatgagaaaggacttgaggccaggcacagtagctaatgtctgtaatgccagcactttgggaagccaaggcagtcagatcacctgaggccaggagttcgagaccagcctggccaacatggtgaaaccctgtctttactaaaaatacaaaaattggctgggcgcggtggctcacgcctgtaatcccagcactttgggaggccaaggcaggcggatcacgaggtcaggagatagagaccatcctggctaacacggtgaaaccctgtctctactaaaaatacaaaaaattagccgggcgtggtggagggcggctgtagtcccagatacttgggaggctgaggcaggagaatggcatgaacccaggaggcggagcttgcagtgagctgagattgcaccactgcactccagcctgggccacagagcgagactccgtctcaaaaaacaatacaaaaattagttgggcatggtggcgagctcctgtaaacccagctactcccaactactagggaggctgaggcaggagaatggcttgaacccagaaggcagaggttacagtgaatcaagataacgccactgcactccaccctgggcgacagagtgagactccgtctcaaaaacaaaaaaataaaaaaaacctcatacactgctggtgggaatataaaatgatgctactactttgaaaagcagtttggcagttcctcaaaaggctaaacatagagttactatatgatgagcactctcacttctaaggtatatgcccagaagaactgaaaacatatatccatataaaaattcatatacgaatattcatagcagcatcatccataatagcaaaaaagtggaaacagtctaaatttcgatcaactgatgaataaactaaatgcggtatatccacacaatagggtattattcagccataaaatgtaatgaagcactggtacactctatagcatagatgaaccttgaaacatgctaagtgaaggaagtcagacacgaaaggccacatgtttatttttataaaatatctagaacaggcaaatcatagagacagaaaatggattattgtttctagaggctgggggaagaggaggattagagtggcagctcactggtatggagtttctaggtagatggaaatgttctggaattagatagtggtgatgattgcacaactctgtaaatatactaaaatccactgcatcatttactttaaaggggcaaattttatggcttgtgaattacatttcaataaaaagaagatgaggaaacctaggatatgtcacaatcccatgccacaaactacttacacttccaatataaaaactatatcaacaatagtttacatcacgttcattgcttgctaaagtaaggtcatgaatgtatcaaaatattttataaaagttaaaatttaggagatccatcatttctcttttcaatccatcactgattcattcaatatatatttatgtgtatgccaggctcttcatcaggtaaagtgtttaggagagatataaagataaaactgatgagaattctgcacttgagctacagcatactttccaagaattacagcatgagatataaaatgaaaagaaggcttggaggagattcacacgaaatagtactgttcaggagagggggcgataattccaatggaagagataactgacttcatggaggatagaaggagatggtatttgaactgcccttgaagtatggttatattttggggatgtggagatgtggggtagggtgatatgctggggttccagatggtccagaaatatacaatcaccagaaccaaagatccagaggtaggagatatgagctgttcaatttggctgagctaacagtgtttggagtgggatcttgaagaagctgaaaatgaagataccaactagacagtcagagaaagacttccaatgtttgactgaactgcaattttattgtgtatgcattgaagaatctttttttttttttttgtattctctaaagatttttaaaatattttaagttctggatacaagtgcaggatgtgcgggtttgttacataggtaaacgtgtcccatggtggtttgctgcacctatcaacctatcacctaggtattaagccccacatgcattagctagttatcctgatgctctccccgctacggcccctgcatcaggccccagtgtgtgttgatctcatccctgtgtccgtgtgttctcattgttcagcttccgcttacaagtgagaacatgtggtgtttggtttcctgctcctctgttagtttgctgaggataatggcttccagcttcatccatgtccctgcaaaggacatgatctcattccttttttaaaaaaaaaaacaaaattatttccataggtgtttggggaacaggtggtatctggttacatgcgtaagtaattaagtggttacttgtgagattctggtgcacccatcacctgagcagtatacactgaacccaatttgtattcttttatccttcacccccctcccaccctttcccctaagtccccaaagtccattgtatccttcttatgcctttgcatcctcatagcttatctcccacttatgagtgagaacatacaatgtttggttttccattcctcagttacttcctttagagtaatagtctccaggttgctgtgaatgtcattaattcattcctttttatggctgagtagtgtttaggtgaggttatttgtaagtaattaatattgagtaaataagattcatccatagtggcaaagccacataacttctaagtatcttaaactatatctaaatggtaccaaaacatgcagtcaattctaaaagctcagctaatgatatttcataatataggaaaatattcacaacatatttttgtgtaaaaaaaagcagacttcaaaatggaatatgcattatgattccaatcatgtaaaagctatacatgaacacatacaaagattaacagatataaacaaatggaagaatgaatggagagatagatgatagacagattgagtggtggtggagaataacagatttaaaaagaaattgtgcctttctatattttcaaaaccatttaaataagtattacctttggagttagaaaatgatatgtattttaaatccataattcaactacttatctatatgatgtcaaactggattaggctgaattatcagcaagtgaataaaacagttccttcatccatggagaaacatccatttatgacattcttggaattcctcttgttagaattctttatgaatttaaaatagaaacatggccagactcaagatttcaatacaaacattactttttcacgttcagtaataaccaattaaaagaattaatgaaaaatctgattcactgtatcaccaaaagctgtaatggctgcactgcacagtattccatggtgtatatgtaccacattttctttatccagtctatctttgatgggcatttgctattgtgtctttgctattgtgaagagtgctgcaatgaacaaaaatgtgcatgtatctttataataaaatggtttatattcctttgggtatatacccagtaatgggattgctgggacaaatagtatttctagttctagatctttgaggaatagccacacacacttccacaacggttgaactaatttacattcccaccaacaatgtaaaagtgttcctacttctccacagcctcgccagcatctgttgttttttgactttttaataatcaccattctgaccggcatgagatggtatctcattgtggttctcctttgcatttctctaatgatcagtaaggttgagcttttttttatatgtttgttggccacataaatgtcttcttttgagaagtgtctgttcatgtcctttgtccactttttgatggggttgtttttttccttgtaaatttgttttaagttccttgtaggttctggatattagacctttgtcagatggatagattgcaaaaatgttctcccattctgtaggttgcctgttcactctaatgatagtttcttttgctgtgcaggagctctttagtttaattagatcccatttgtaatttttgcttttgttgcaattgcttttgatgtttttgtcatgaaacctttgcttgtgcctatgtcttgaatggtattaaatagattttcttctagggtttttatagttttaggttttacattaagtctttaatcttgagttaatttttgtataaggtgtaaggaaggggtcagtttcaattttctgcatatggctagccagttttcccagcaccatttattaaatagggaatcttttccccattgcttgtttttgtcaggtttgtcgatgatcagatggctgtagatgtgtggtcttctttctctggtctctattctgttccattggtctatgtgtctgtttttgtaccagtaccatgccattttggctactgtagccttgcagtatactttgaagttgggtagtgtgatgcttccagctttgttctttttgcttattgttgtcttggttatacgggctcttttttggttccatttgaattttaaagtagtttttttctaattctgtgaagaatgtcaatagtagtttaatgggaatagcaatgaacctataaattactttgggtagtatggccattttcatgatattgattcttcctatccacgagaatggaatgttttttcatttgtgtcctctcttatttccttgagcagtggtttgtagttctccttgaagagatccttcacatcttattagctgtattcctaggtattttattctctttctagcaactgtgaatgggagttcattcatgatttggctctctgcttgtgtattgttggtgtatagaatgcttgtgatttctgcacattgattttgtatcctgagactttgctgaagttgcttatcagcttaaggaacttttgggtggagataatggggttttctagatatagtatcatgtcatctgcaaacacagttttacttcctcttttcctatttgaataccccttatttgtttctcttgcctgattttcttggccagaacttccaatactatgttaaataggagtggtgagacggcatccctgtcttgtgccagttttcaaggggaatgcttccagcttttgcccattcagtatgataatggctgtgggtttgtcataaatggttattattttgagatattttccatcaatacctagtttattgagagtttttaacatgaagcaacgttgaattttattgaaggccttttctgtatctattgagataatcatgtggtttttgtctttagttctgtttatgtgatgaattatgtttcttgatttgcgtatgttgaaccagccttgcatcccagggatgaagccaacattccaaacattttatttattatttatttatttatttatttttgagacagagtctcgcactgtcgcccaggctggagtgcagtggcaagatctcagctcgctgcaagctccacctcccaggttcatgccgttctcttgcctcggcctcccaaatagcagggactacaggcgaccgccacaacgcctggctaattttttgtatttttagtagagacggggttttacatgttagccaggatggtcttgatctcctgacctcgtgatccgcccgccttggcctcccaaagggctgggattataggcgtgagccaccgcacccggcctccaaacattttaatctcataacaatgcatcacttgggttaactaggttgagataaatataaactgtcaattttttttcccctcacataaaagtccagaggtaggtaattagggctgacacagtgattccagtgattctgctccttcgtgccctcatccaacaaggcttcttgctgctcactacccagctacccctacgtgtggcccgtatcttcatggttcaagatggcagctagagctgctaggtagttaagatctctctcacacactttccttctgtcataattaacacagggttttagctcatgaggccaagcatacacattacttcccactggcacccctatgtaatattaaatgcaaagataccctcaggagtcctgtgctcaaaacaagtacaaaataactttttgttgttgtttgtggtgctggtggttttatttatttattttttctgaaacagggtctcactctgtctcccatgctgaagtgcagtggtgtgatcacagctcatcacaaccttgacctctctgggctcaggggatccactcacttcagcctcccaagtagctgggactacaggaacacgccaccacgctcagctaaattttgtctttttttgtagagatggagtcttgctatgttgcccaggctggtctcaaactcctgggctcaagtgatcagtccacctcagcctcccaaagtactcagattataggtatgagccaccatggcatcaaaataacttggaaagtaggaataattgcttgttgttcctgaaaactgtctcttcgacacttttcagactctgttacatgatcatgacaaaatatacacaaatagacatacagatacacatcagttaaaacctcaagaaatagaaaaataaataaatcataaaatatttaaaaagtggtattctgacacactgcccagaggtacccctgttcagcaattttaaaaaattttaaaaatagccctctccccctccctctcttctccctctccccacggtctccctctgatgccgagccgaagctggactgtactgctgccatctcggctcactgcagcctccctgcctgattctcccgcctcggcctgccgcgtgcctgccattgcgggcgccgccacgcctgactggttttcgtatttttttggtggagacagggtttcactgtgttggccgggctggtctccagctcctgactgcgagtgatctgccagcctcggcctcccgaggtgccgggattgcgggcagagtctcgtccactcagtgctcaatgttgcccaggctggagtgcagtggtgtgatctcagctggctacggcctccgcctcccagccgcctgccttggccccccagggtgccgagattacagcttctgcccggccgccaccccgtctgggatgaagtgaggagcgtctctgcccggccgcccatcgtctgagatgtggggagcgcctctgccccgcccccccgtctgggatgtgaggagcttctctgcccggccaccccgtctgagaagtgaggagcccctccgcccgcagctgccccgtctgagaagtgaggagcccctccgcccgacagccaccctgtctgggaagtgaggagcgtctccgcccagcagccaccccgtctgagaagtgaggagcccctccgcctggcagccgccccgtccgggagggaggcgtgggggtcagcccccgcccggccagccgccccgtcggggagggaggtggggggtcagcccccgcccggccagctatcccgtccgggagggaggtggggggcgcgtccgcctggccgccccatctgggaagtgaggagcccctctgcccagccgccaccccgtctgggaggtgtacccaacagctcattgagaacaggccatgatgacgatggcggttttgtggaatagaaaagggggaaaggtggggaaaagatagagaaatcagattgttgctgtgtctgtgtagaaagaagtagacatgggagacttcattttgttctgtactaagaaaaattcttctgccttaggatgctgttgatctatgaccttacccccaaccctgtgctctctgaaacatgtgctgtgtccactcagggttaaatggattaagggcagtgcaagatgtgctttgttaaacagatgcttgaaggcagcatgctccttaagagtcatcaccactccctaatctcaagtacccagggacacaaacactgcggaaggccgcagggtcctctgcctaggaaaaccagagacctttgttcacttgtttatctgctgaccttccctccactattgtcctgtgaccctgccaaatcaccctctgtgagaaacacccaagaatgatcaattaaaaaaaaaaaatttaaaaataataataggccaggtgcagtggctcacacctgtaatcccagcactttgggaggccgaggctggtgaatcacctgaggtcaggagttcaagaccacgctggccaacatggtggaaaccctgtctccactaaaaatacaaaaattagccgggtgtggtggcaggagcctgtaatcccagctactcgggaggctgaggcaggagaatcgcttgaacccagaaggcagaggttgcaatgagccaagatgatgccactgcactccagcctgggcagcagaatgaaactctgtctcaataataataataataataataataataataataataataataataagcaactctaatgatatttcaaacaatggtccccttttaggtcacactatcaaatcagagaaagatatacttgactagctgtaaaatgcaatttgaggtctaggtgaatgaacaagtaacctctaaatcataaggctattgttacaaactgaatgtttgtattccccccagaattcaaaggggagacagtatccccaaagtgacagtatcagaaggtggggcctttgggaggtaattaggtgatgagggtagagccctcatgaatggaatttgtgcccttaaagatatacttgagagtttgcatcctctttttctgccatgtgagaacatcaaaagactgacatctggtaagatctggaagcatgccttaccagacaccagatatgctaccacttagatgttggatttcccagcctccggaactgtgagaaataactgctgtttaagtcacctggtctatggtaatttggtatagttgcccaaatggactgtgatggttaatactgagtatcaacttgattgaatagaaggatgcaaagtgttcccgggtacatctgtgagggtgctgccaaaggagatttaacatttgagtcagtggactgggaaaggcagaccatcctcaatctgggtgggcaccatctaatcagctgccagcactgccagaataaaagcaggcaaaacatggaaagactagactggtgtagtcttctggcctccatctttctctcatgctgaatgcttcctgccctcaaacattggactccaagttcttcagctttgggacttgaattggcttccttgcttgcagatgacctattgtgggacctaaccctgtgatcatgtgagtcaatactccttaataaactcccctttttatatacatgtatcctattagttctgtccctctagagaaacatgactaatacattgagtaagatagttcctgtcctttttttttttttttaaagagatgggatcttgctatattgcccaggttggtatgcagtggctattcgtaggcacaatcacagcatgctatgaccctgaactcctgggttcaaaagatcctcccacctcagcctcccaagtaactgggaatacaggtacccacacccacacccagctaatttttgtatttttactagggacagcgtttaccatgttggccaggctggtctcgaactcctgacctgaagtgatctgccctccttggcctcccaaagtgctgggattacaggtgtgagccactacgcccagccttttggtttcttatgtgtaggagaggataagtttctttctcagagtgtgctgcagccagacataatatttctccttggcagaaactctgctgttccaatcatacatgtagccattgagttcaatgtgaagatccaggagtgggcgttttctttcttgtctcagtttctgggagaggcactgcaggtacagggatggtgagctgtgagactgctccagcagggacatgtccgcagtacacaggctccagaagaagtcagcttctcggtgaactgtgcacagccctcgcttctgagccttgaattccacattcttcatcgctggcccatccacctccaagaggctgctgtcctccagctggccctctgacaccacatagttctgaataaaaaacatctttggcttccctgctagataagggcatgaatctcccatgaacatcctcctgatgtgatgcagggggagccctgagtgagtctgatccacaccatacacactctgggagcctcctcggctcaccaggacacacacaaagctgtcgtagtctcggtgctcgggcatacaggcaaattggccaagaatctgggatataccatgcatactgagatgcaagaatttctggacttcatagcccagggaagtgaaggtgtctcgaagaagctctgtctcattgccaatgcaatcgattatcaggcagattcctaggggcttgctcttcatcttgtatctctcttcaggtatgctctgaggcaaaaaagcttctgattcctgaatggatttcttcactggttcttgttgagcgccaagctgttccttaagtctttgttctttacttctcccattatggagcctgaagttatttgaaggatccttgagactcttttggattgctgcttggagaacattcctgtaacttgtccctgctccttgaacagactgcttgtacttctggatttttgtcttcaggtctattctgtggatgttctttaggcatttttctaataaatccagttgatctggggcaaccagatttagtttctccaactcaaccacaaggtccaagaaactcttctccttgcttatcttgcctcggcccatgtaatccttcatgaggaaaattaatgaggacacatcagatttatccaaatcctcaccaatctctgccatcagcactctatagtccgaaacaaggtgagggttcctgagcaggtgggtctccacagcttttctgtccatcttcaagatacgtttgagcaggtcaaatcgcctcactctgtagagcagttcagccaagtccccgacagacagcttacctctttcccgtaaaatatccagaaggtccctgacattaggtggaaccacatctatagcaacatcccggcacaaaaagagcagcatctccttctcatctgtatcaagtgcttcttcaacctgatggatgacttcagcagacatcctactcttagactagggaagctcacaagggtcttgcagtacagctccgggccagtcaacagaaagccagcaggcagtcaacttcatttctgagggctgacttcatttctttcagaatcctttccagtgggggagttgcccgggcagccgccggctcttcccactggatctccgccgggaccaactcccaccctcgccggacaagctcagacctgctgctccgcaaaaccagaattggaaatgctccagatgggacgaggaacaaggacagaaagtcaaaagcatcaacaggtggcttcgccggagggcgtccgagaacctct

SEQ ID NO: 15269 - RNA, 13030 nt, Homo sapiens
  source 1..13030: mol_type = other RNA
gctgggattacaggcatgagccactgcgcccagccaaacttatctttgtatgtttgttataggcaaaagtaccccaaggttaaggctcagcccaagaggtcaagtgggttcaggaaagaattcaagagcatgctgacagaataaagtgaaagcaagttcattaagaaagtaaaggaataaaagaatggctaccccataggaagagtagccctgatgggctgctgactggctatatttatggttgcttcttgactatacgctaaacaagaggtggcttattcatgagttttccaggaaagaagtggggaggtctggaccttttagaccatacagggtaacttctgaaagttgctatggcagttgtaaactatcatggtgctgtagaagtttcttttagcgtgctaatgtattataattaccatagaatgggcagcaaaggtaaccagaggtctcttctgtcaccatcatggttttggctggtttgggttggcctttctaccacatcctgtcttatcagcagggtcttacagggtcttgtggtcttgggaaaccagtcctgccaaactcctctcattcagtgtaatcactatcaaaattccagaggccctttttacataaatttgcaagtgaatcctaacagttatatgaaaatttagggaaaggtaaacccaatacagccctaacaattttgaaaaagaacaggccagttgcagtggctcacccctcagcactttgggaggtggaggtgggaggattgtttgaggccaggagtttgagaccagcctgggcaacatagcaaggcctcatctctacaaaagaaaaaagaagaacaacaacaacaacaaagttagaggactacatttctggattccaaaacttactacgaagttacaataatcaagacagtgtggtactaccataagatagagcaacagaattgagtccagaaataaacccttatagttagttgatttgtgataagtataaaataattctatagggaaaaaatagtattttcaataagtaatgctaagacaagtgaacatttatgtgcaaaagaatgaggctggatgcttatctcgcactgcatacacaaaaataactcaaaatgggtcaaagagctaaaatcataaaactttagaagaaaacataggggtaacacctcataggcaattgatttagacaatggttttttaggtatgacaccaaaagcataagcaataacataaaaaacagaaatcaagtgaacttcatcaaaatttaaaacttgtactgtatagtatccagaaagtgagaagacaatccatggaatgggagaatatattcacaaagattgtacctgataagaaactagtatccagaatattaaaaagaatgcttacaactcaacaataaaaagacaacccaccgggtgtggtggctcacgcctgtaatcctagcattttgggaggccgaggcaggcagatcacctgagttcaggagttcaagaccagcctggccaacatggcgaaaccctgtctctactaaaaatacaaaaattagccaggcgtgatggtgggtgcctgtaatcccagttactagggaggccgaggcaggagagtcgcttgaactcaggaggtggaggttgcagtgagccgagattgcaccactgcactccaacctgggcgacagagtgagattccatctcagaaaaataaaataaaataacgcagttttaaaatgagaaaggacttgaggccaggcacagtagctaatgtctgtaatgccagcactttgggaagccaaggcagtcagatcacctgaggccaggagttcgagaccagcctggccaacatggtgaaaccctgtctttactaaaaatacaaaaattggctgggcgcggtggctcacgcctgtaatcccagcactttgggaggccaaggcaggcggatcacgaggtcaggagatagagaccatcctggctaacacggtgaaaccctgtctctactaaaaatacaaaaaattagccgggcgtggtggagggcggctgtagtcccagatacttgggaggctgaggcaggagaatggcatgaacccaggaggcggagcttgcagtgagctgagattgcaccactgcactccagcctgggccacagagcgagactccgtctcaaaaaacaatacaaaaattagttgggcatggtggcgagctcctgtaaacccagctactcccaactactagggaggctgaggcaggagaatggcttgaacccagaaggcagaggttacagtgaatcaagataacgccactgcactccaccctgggcgacagagtgagactccgtctcaaaaacaaaaaaataaaaaaaacctcatacactgctggtgggaatataaaatgatgctactactttgaaaagcagtttggcagttcctcaaaaggctaaacatagagttactatatgatgagcactctcacttctaaggtatatgcccagaagaactgaaaacatatatccatataaaaattcatatacgaatattcatagcagcatcatccataatagcaaaaaagtggaaacagtctaaatttcgatcaactgatgaataaactaaatgcggtatatccacacaatagggtattattcagccataaaatgtaatgaagcactggtacactctatagcatagatgaaccttgaaacatgctaagtgaaggaagtcagacacgaaaggccacatgtttatttttataaaatatctagaacaggcaaatcatagagacagaaaatggattattgtttctagaggctgggggaagaggaggattagagtggcagctcactggtatggagtttctaggtagatggaaatgttctggaattagatagtggtgatgattgcacaactctgtaaatatactaaaatccactgcatcatttactttaaaggggcaaattttatggcttgtgaattacatttcaataaaaagaagatgaggaaacctaggatatgtcacaatcccatgccacaaactacttacacttccaatataaaaactatatcaacaatagtttacatcacgttcattgcttgctaaagtaaggtcatgaatgtatcaaaatattttataaaagttaaaatttaggagatccatcatttctcttttcaatccatcactgattcattcaatatatatttatgtgtatgccaggctcttcatcaggtaaagtgtttaggagagatataaagataaaactgatgagaattctgcacttgagctacagcatactttccaagaattacagcatgagatataaaatgaaaagaaggcttggaggagattcacacgaaatagtactgttcaggagagggggcgataattccaatggaagagataactgacttcatggaggatagaaggagatggtatttgaactgcccttgaagtatggttatattttggggatgtggagatgtggggtagggtgatatgctggggttccagatggtccagaaatatacaatcaccagaaccaaagatccagaggtaggagatatgagctgttcaatttggctgagctaacagtgtttggagtgggatcttgaagaagctgaaaatgaagataccaactagacagtcagagaaagacttccaatgtttgactgaactgcaattttattgtgtatgcattgaagaatctttttttttttttttgtattctctaaagatttttaaaatattttaagttctggatacaagtgcaggatgtgcgggtttgttacataggtaaacgtgtcccatggtggtttgctgcacctatcaacctatcacctaggtattaagccccacatgcattagctagttatcctgatgctctccccgctacggcccctgcatcaggccccagtgtgtgttgatctcatccctgtgtccgtgtgttctcattgttcagcttccgcttacaagtgagaacatgtggtgtttggtttcctgctcctctgttagtttgctgaggataatggcttccagcttcatccatgtccctgcaaaggacatgatctcattccttttttaaaaaaaaaaacaaaattatttccataggtgtttggggaacaggtggtatctggttacatgcgtaagtaattaagtggttacttgtgagattctggtgcacccatcacctgagcagtatacactgaacccaatttgtattcttttatccttcacccccctcccaccctttcccctaagtccccaaagtccattgtatccttcttatgcctttgcatcctcatagcttatctcccacttatgagtgagaacatacaatgtttggttttccattcctcagttacttcctttagagtaatagtctccaggttgctgtgaatgtcattaattcattcctttttatggctgagtagtgtttaggtgaggttatttgtaagtaattaatattgagtaaataagattcatccatagtggcaaagccacataacttctaagtatcttaaactatatctaaatggtaccaaaacatgcagtcaattctaaaagctcagctaatgatatttcataatataggaaaatattcacaacatatttttgtgtaaaaaaaagcagacttcaaaatggaatatgcattatgattccaatcatgtaaaagctatacatgaacacatacaaagattaacagatataaacaaatggaagaatgaatggagagatagatgatagacagattgagtggtggtggagaataacagatttaaaaagaaattgtgcctttctatattttcaaaaccatttaaataagtattacctttggagttagaaaatgatatgtattttaaatccataattcaactacttatctatatgatgtcaaactggattaggctgaattatcagcaagtgaataaaacagttccttcatccatggagaaacatccatttatgacattcttggaattcctcttgttagaattctttatgaatttaaaatagaaacatggccagactcaagatttcaatacaaacattactttttcacgttcagtaataaccaattaaaagaattaatgaaaaatctgattcactgtatcaccaaaagctgtaatggctgcactgcacagtattccatggtgtatatgtaccacattttctttatccagtctatctttgatgggcatttgctattgtgtctttgctattgtgaagagtgctgcaatgaacaaaaatgtgcatgtatctttataataaaatggtttatattcctttgggtatatacccagtaatgggattgctgggacaaatagtatttctagttctagatctttgaggaatagccacacacacttccacaacggttgaactaatttacattcccaccaacaatgtaaaagtgttcctacttctccacagcctcgccagcatctgttgttttttgactttttaataatcaccattctgaccggcatgagatggtatctcattgtggttctcctttgcatttctctaatgatcagtaaggttgagcttttttttatatgtttgttggccacataaatgtcttcttttgagaagtgtctgttcatgtcctttgtccactttttgatggggttgtttttttccttgtaaatttgttttaagttccttgtaggttctggatattagacctttgtcagatggatagattgcaaaaatgttctcccattctgtaggttgcctgttcactctaatgatagtttcttttgctgtgcaggagctctttagtttaattagatcccatttgtaatttttgcttttgttgcaattgcttttgatgtttttgtcatgaaacctttgcttgtgcctatgtcttgaatggtattaaatagattttcttctagggtttttatagttttaggttttacattaagtctttaatcttgagttaatttttgtataaggtgtaaggaaggggtcagtttcaattttctgcatatggctagccagttttcccagcaccatttattaaatagggaatcttttccccattgcttgtttttgtcaggtttgtcgatgatcagatggctgtagatgtgtggtcttctttctctggtctctattctgttccattggtctatgtgtctgtttttgtaccagtaccatgccattttggctactgtagccttgcagtatactttgaagttgggtagtgtgatgcttccagctttgttctttttgcttattgttgtcttggttatacgggctcttttttggttccatttgaattttaaagtagtttttttctaattctgtgaagaatgtcaatagtagtttaatgggaatagcaatgaacctataaattactttgggtagtatggccattttcatgatattgattcttcctatccacgagaatggaatgttttttcatttgtgtcctctcttatttccttgagcagtggtttgtagttctccttgaagagatccttcacatcttattagctgtattcctaggtattttattctctttctagcaactgtgaatgggagttcattcatgatttggctctctgcttgtgtattgttggtgtatagaatgcttgtgatttctgcacattgattttgtatcctgagactttgctgaagttgcttatcagcttaaggaacttttgggtggagataatggggttttctagatatagtatcatgtcatctgcaaacacagttttacttcctcttttcctatttgaataccccttatttgtttctcttgcctgattttcttggccagaacttccaatactatgttaaataggagtggtgagacggcatccctgtcttgtgccagttttcaaggggaatgcttccagcttttgcccattcagtatgataatggctgtgggtttgtcataaatggttattattttgagatattttccatcaatacctagtttattgagagtttttaacatgaagcaacgttgaattttattgaaggccttttctgtatctattgagataatcatgtggtttttgtctttagttctgtttatgtgatgaattatgtttcttgatttgcgtatgttgaaccagccttgcatcccagggatgaagccaacattccaaacattttatttattatttatttatttatttatttttgagacagagtctcgcactgtcgcccaggctggagtgcagtggcaagatctcagctcgctgcaagctccacctcccaggttcatgccgttctcttgcctcggcctcccaaatagcagggactacaggcgaccgccacaacgcctggctaattttttgtatttttagtagagacggggttttacatgttagccaggatggtcttgatctcctgacctcgtgatccgcccgccttggcctcccaaagggctgggattataggcgtgagccaccgcacccggcctccaaacattttaatctcataacaatgcatcacttgggttaactaggttgagataaatataaactgtcaattttttttcccctcacataaaagtccagaggtaggtaattagggctgacacagtgattccagtgattctgctccttcgtgccctcatccaacaaggcttcttgctgctcactacccagctacccctacgtgtggcccgtatcttcatggttcaagatggcagctagagctgctaggtagttaagatctctctcacacactttccttctgtcataattaacacagggttttagctcatgaggccaagcatacacattacttcccactggcacccctatgtaatattaaatgcaaagataccctcaggagtcctgtgctcaaaacaagtacaaaataactttttgttgttgtttgtggtgctggtggttttatttatttattttttctgaaacagggtctcactctgtctcccatgctgaagtgcagtggtgtgatcacagctcatcacaaccttgacctctctgggctcaggggatccactcacttcagcctcccaagtagctgggactacaggaacacgccaccacgctcagctaaattttgtctttttttgtagagatggagtcttgctatgttgcccaggctggtctcaaactcctgggctcaagtgatcagtccacctcagcctcccaaagtactcagattataggtatgagccaccatggcatcaaaataacttggaaagtaggaataattgcttgttgttcctgaaaactgtctcttcgacacttttcagactctgttacatgatcatgacaaaatatacacaaatagacatacagatacacatcagttaaaacctcaagaaatagaaaaataaataaatcataaaatatttaaaaagtggtattctgacacactgcccagaggtacccctgttcagcaattttaaaaaattttaaaaatagccctctccccctccctctcttctccctctccccacggtctccctctgatgccgagccgaagctggactgtactgctgccatctcggctcactgcagcctccctgcctgattctcccgcctcggcctgccgcgtgcctgccattgcgggcgccgccacgcctgactggttttcgtatttttttggtggagacagggtttcactgtgttggccgggctggtctccagctcctgactgcgagtgatctgccagcctcggcctcccgaggtgccgggattgcgggcagagtctcgtccactcagtgctcaatgttgcccaggctggagtgcagtggtgtgatctcagctggctacggcctccgcctcccagccgcctgccttggccccccagggtgccgagattacagcttctgcccggccgccaccccgtctgggatgaagtgaggagcgtctctgcccggccgcccatcgtctgagatgtggggagcgcctctgccccgcccccccgtctgggatgtgaggagcttctctgcccggccaccccgtctgagaagtgaggagcccctccgcccgcagctgccccgtctgagaagtgaggagcccctccgcccgacagccaccctgtctgggaagtgaggagcgtctccgcccagcagccaccccgtctgagaagtgaggagcccctccgcctggcagccgccccgtccgggagggaggcgtgggggtcagcccccgcccggccagccgccccgtcggggagggaggtggggggtcagcccccgcccggccagctatcccgtccgggagggaggtggggggcgcgtccgcctggccgccccatctgggaagtgaggagcccctctgcccagccgccaccccgtctgggaggtgtacccaacagctcattgagaacaggccatgatgacgatggcggttttgtggaatagaaaagggggaaaggtggggaaaagatagagaaatcagattgttgctgtgtctgtgtagaaagaagtagacatgggagacttcattttgttctgtactaagaaaaattcttctgccttaggatgctgttgatctatgaccttacccccaaccctgtgctctctgaaacatgtgctgtgtccactcagggttaaatggattaagggcagtgcaagatgtgctttgttaaacagatgcttgaaggcagcatgctccttaagagtcatcaccactccctaatctcaagtacccagggacacaaacactgcggaaggccgcagggtcctctgcctaggaaaaccagagacctttgttcacttgtttatctgctgaccttccctccactattgtcctgtgaccctgccaaatcaccctctgtgagaaacacccaagaatgatcaattaaaaaaaaaaaatttaaaaataataataggccaggtgcagtggctcacacctgtaatcccagcactttgggaggccgaggctggtgaatcacctgaggtcaggagttcaagaccacgctggccaacatggtggaaaccctgtctccactaaaaatacaaaaattagccgggtgtggtggcaggagcctgtaatcccagctactcgggaggctgaggcaggagaatcgcttgaacccagaaggcagaggttgcaatgagccaagatgatgccactgcactccagcctgggcagcagaatgaaactctgtctcaataataataataataataataataataataataataataataataagcaactctaatgatatttcaaacaatggtccccttttaggtcacactatcaaatcagagaaagatatacttgactagctgtaaaatgcaatttgaggtctaggtgaatgaacaagtaacctctaaatcataaggctattgttacaaactgaatgtttgtattccccccagaattcaaaggggagacagtatccccaaagtgacagtatcagaaggtggggcctttgggaggtaattaggtgatgagggtagagccctcatgaatggaatttgtgcccttaaagatatacttgagagtttgcatcctctttttctgccatgtgagaacatcaaaagactgacatctggtaagatctggaagcatgccttaccagacaccagatatgctaccacttagatgttggatttcccagcctccggaactgtgagaaataactgctgtttaagtcacctggtctatggtaatttggtatagttgcccaaatggactgtgatggttaatactgagtatcaacttgattgaatagaaggatgcaaagtgttcccgggtacatctgtgagggtgctgccaaaggagatttaacatttgagtcagtggactgggaaaggcagaccatcctcaatctgggtgggcaccatctaatcagctgccagcactgccagaataaaagcaggcaaaacatggaaagactagactggtgtagtcttctggcctccatctttctctcatgctgaatgcttcctgccctcaaacattggactccaagttcttcagctttgggacttgaattggcttccttgcttgcagatgacctattgtgggacctaaccctgtgatcatgtgagtcaatactccttaataaactcccctttttatatacatgtatcctattagttctgtccctctagagaaacatgactaatacattgagtaagatagttcctgtcctttttttttttttttaaagagatgggatcttgctatattgcccaggttggtatgcagtggctattcgtaggcacaatcacagcatgctatgaccctgaactcctgggttcaaaagatcctcccacctcagcctcccaagtaactgggaatacaggtacccacacccacacccagctaatttttgtatttttactagggacagcgtttaccatgttggccaggctggtctcgaactcctgacctgaagtgatctgccctccttggcctcccaaagtgctgggattacaggtgtgagccactacgcccagccttttggtttcttatgtgtaggagaggataagtttctttctcagagtgtgctgcagccagacataatatttctccttggcagaaactctgctgttccaatcatacatgtagccattgagttcaatgtgaagatccaggagtgggcgttttctttcttgtctcagtttctgggagaggcactgcaggtacagggatggtgagctgtgagactgctccagcagggacatgtccgcagtacacaggctccagaagaagtcagcttctcggtgaactgtgcacagccctcgcttctgagccttgaattccacattcttcatcgctggcccatccacctccaagaggctgctgtcctccagctggccctctgacaccacatagttctgaataaaaaacatctttggcttccctgctagataagggcatgaatctcccatgaacatcctcctgatgtgatgcagggggagccctgagtgagtctgatccacaccatacacactctgggagcctcctcggctcaccaggacacacacaaagctgtcgtagtctcggtgctcgggcatacaggcaaattggccaagaatctgggatataccatgcatactgagatgcaagaatttctggacttcatagcccagggaagtgaaggtgtctcgaagaagctctgtctcattgccaatgcaatcgattatcaggcagattcctaggggcttgctcttcatcttgtatctctcttcaggtatgctctgaggcaaaaaagcttctgattcctgaatggatttcttcactggttcttgttgagcgccaagctgttccttaagtctttgttctttacttctcccattatggagcctgaagttatttgaaggatccttgagactcttttggattgctgcttggagaacattcctgtaacttgtccctgctccttgaacagactgcttgtacttctggatttttgtcttcaggtctattctgtggatgttctttaggcatttttctaataaatccagttgatctggggcaaccagatttagtttctccaactcaaccacaaggtccaagaaactcttctccttgcttatcttgcctcggcccatgtaatccttcatgaggaaaattaatgaggacacatcagatttatccaaatcctcaccaatctctgccatcagcactctctttcccgtaaaatatccagaaggtccctgacattaggtggaaccacatctatagcaacatcccggcacaaaaagagcagcatctccttctcatctgtatcaagtgcttcttcaacctgatggatgacttcagcagacatcctactcttagactagggaagctcacaagggtcttgcagtacagctccgggccagtcaacagaaagccagcaggcagtcaacttcatttctgagggctgacttcatttctttcagaatcctttccagtgggggagttgcccgggcagccgccggctcttcccactggatctccgccgggaccaactcccaccctcgccggacaagctcagacctgctgctccgcaaaaccagaattggaaatgctccagatgggacgaggaacaaggacagaaagtcaaaagcatcaacaggtggcttcgccggagggcgtccgagaacctct

SEQ ID NO: 15270 - RNA, 12751 nt, Homo sapiens
  source 1..12751: mol_type = other RNA
gctgggattacaggcatgagccactgcgcccagccaaacttatctttgtatgtttgttataggcaaaagtaccccaaggttaaggctcagcccaagaggtcaagtgggttcaggaaagaattcaagagcatgctgacagaataaagtgaaagcaagttcattaagaaagtaaaggaataaaagaatggctaccccataggaagagtagccctgatgggctgctgactggctatatttatggttgcttcttgactatacgctaaacaagaggtggcttattcatgagttttccaggaaagaagtggggaggtctggaccttttagaccatacagggtaacttctgaaagttgctatggcagttgtaaactatcatggtgctgtagaagtttcttttagcgtgctaatgtattataattaccatagaatgggcagcaaaggtaaccagaggtctcttctgtcaccatcatggttttggctggtttgggttggcctttctaccacatcctgtcttatcagcagggtcttacagggtcttgtggtcttgggaaaccagtcctgccaaactcctctcattcagtgtaatcactatcaaaattccagaggccctttttacataaatttgcaagtgaatcctaacagttatatgaaaatttagggaaaggtaaacccaatacagccctaacaattttgaaaaagaacaggccagttgcagtggctcacccctcagcactttgggaggtggaggtgggaggattgtttgaggccaggagtttgagaccagcctgggcaacatagcaaggcctcatctctacaaaagaaaaaagaagaacaacaacaacaacaaagttagaggactacatttctggattccaaaacttactacgaagttacaataatcaagacagtgtggtactaccataagatagagcaacagaattgagtccagaaataaacccttatagttagttgatttgtgataagtataaaataattctatagggaaaaaatagtattttcaataagtaatgctaagacaagtgaacatttatgtgcaaaagaatgaggctggatgcttatctcgcactgcatacacaaaaataactcaaaatgggtcaaagagctaaaatcataaaactttagaagaaaacataggggtaacacctcataggcaattgatttagacaatggttttttaggtatgacaccaaaagcataagcaataacataaaaaacagaaatcaagtgaacttcatcaaaatttaaaacttgtactgtatagtatccagaaagtgagaagacaatccatggaatgggagaatatattcacaaagattgtacctgataagaaactagtatccagaatattaaaaagaatgcttacaactcaacaataaaaagacaacccaccgggtgtggtggctcacgcctgtaatcctagcattttgggaggccgaggcaggcagatcacctgagttcaggagttcaagaccagcctggccaacatggcgaaaccctgtctctactaaaaatacaaaaattagccaggcgtgatggtgggtgcctgtaatcccagttactagggaggccgaggcaggagagtcgcttgaactcaggaggtggaggttgcagtgagccgagattgcaccactgcactccaacctgggcgacagagtgagattccatctcagaaaaataaaataaaataacgcagttttaaaatgagaaaggacttgaggccaggcacagtagctaatgtctgtaatgccagcactttgggaagccaaggcagtcagatcacctgaggccaggagttcgagaccagcctggccaacatggtgaaaccctgtctttactaaaaatacaaaaattggctgggcgcggtggctcacgcctgtaatcccagcactttgggaggccaaggcaggcggatcacgaggtcaggagatagagaccatcctggctaacacggtgaaaccctgtctctactaaaaatacaaaaaattagccgggcgtggtggagggcggctgtagtcccagatacttgggaggctgaggcaggagaatggcatgaacccaggaggcggagcttgcagtgagctgagattgcaccactgcactccagcctgggccacagagcgagactccgtctcaaaaaacaatacaaaaattagttgggcatggtggcgagctcctgtaaacccagctactcccaactactagggaggctgaggcaggagaatggcttgaacccagaaggcagaggttacagtgaatcaagataacgccactgcactccaccctgggcgacagagtgagactccgtctcaaaaacaaaaaaataaaaaaaacctcatacactgctggtgggaatataaaatgatgctactactttgaaaagcagtttggcagttcctcaaaaggctaaacatagagttactatatgatgagcactctcacttctaaggtatatgcccagaagaactgaaaacatatatccatataaaaattcatatacgaatattcatagcagcatcatccataatagcaaaaaagtggaaacagtctaaatttcgatcaactgatgaataaactaaatgcggtatatccacacaatagggtattattcagccataaaatgtaatgaagcactggtacactctatagcatagatgaaccttgaaacatgctaagtgaaggaagtcagacacgaaaggccacatgtttatttttataaaatatctagaacaggcaaatcatagagacagaaaatggattattgtttctagaggctgggggaagaggaggattagagtggcagctcactggtatggagtttctaggtagatggaaatgttctggaattagatagtggtgatgattgcacaactctgtaaatatactaaaatccactgcatcatttactttaaaggggcaaattttatggcttgtgaattacatttcaataaaaagaagatgaggaaacctaggatatgtcacaatcccatgccacaaactacttacacttccaatataaaaactatatcaacaatagtttacatcacgttcattgcttgctaaagtaaggtcatgaatgtatcaaaatattttataaaagttaaaatttaggagatccatcatttctcttttcaatccatcactgattcattcaatatatatttatgtgtatgccaggctcttcatcaggtaaagtgtttaggagagatataaagataaaactgatgagaattctgcacttgagctacagcatactttccaagaattacagcatgagatataaaatgaaaagaaggcttggaggagattcacacgaaatagtactgttcaggagagggggcgataattccaatggaagagataactgacttcatggaggatagaaggagatggtatttgaactgcccttgaagtatggttatattttggggatgtggagatgtggggtagggtgatatgctggggttccagatggtccagaaatatacaatcaccagaaccaaagatccagaggtaggagatatgagctgttcaatttggctgagctaacagtgtttggagtgggatcttgaagaagctgaaaatgaagataccaactagacagtcagagaaagacttccaatgtttgactgaactgcaattttattgtgtatgcattgaagaatctttttttttttttttgtattctctaaagatttttaaaatattttaagttctggatacaagtgcaggatgtgcgggtttgttacataggtaaacgtgtcccatggtggtttgctgcacctatcaacctatcacctaggtattaagccccacatgcattagctagttatcctgatgctctccccgctacggcccctgcatcaggccccagtgtgtgttgatctcatccctgtgtccgtgtgttctcattgttcagcttccgcttacaagtgagaacatgtggtgtttggtttcctgctcctctgttagtttgctgaggataatggcttccagcttcatccatgtccctgcaaaggacatgatctcattccttttttaaaaaaaaaaacaaaattatttccataggtgtttggggaacaggtggtatctggttacatgcgtaagtaattaagtggttacttgtgagattctggtgcacccatcacctgagcagtatacactgaacccaatttgtattcttttatccttcacccccctcccaccctttcccctaagtccccaaagtccattgtatccttcttatgcctttgcatcctcatagcttatctcccacttatgagtgagaacatacaatgtttggttttccattcctcagttacttcctttagagtaatagtctccaggttgctgtgaatgtcattaattcattcctttttatggctgagtagtgtttaggtgaggttatttgtaagtaattaatattgagtaaataagattcatccatagtggcaaagccacataacttctaagtatcttaaactatatctaaatggtaccaaaacatgcagtcaattctaaaagctcagctaatgatatttcataatataggaaaatattcacaacatatttttgtgtaaaaaaaagcagacttcaaaatggaatatgcattatgattccaatcatgtaaaagctatacatgaacacatacaaagattaacagatataaacaaatggaagaatgaatggagagatagatgatagacagattgagtggtggtggagaataacagatttaaaaagaaattgtgcctttctatattttcaaaaccatttaaataagtattacctttggagttagaaaatgatatgtattttaaatccataattcaactacttatctatatgatgtcaaactggattaggctgaattatcagcaagtgaataaaacagttccttcatccatggagaaacatccatttatgacattcttggaattcctcttgttagaattctttatgaatttaaaatagaaacatggccagactcaagatttcaatacaaacattactttttcacgttcagtaataaccaattaaaagaattaatgaaaaatctgattcactgtatcaccaaaagctgtaatggctgcactgcacagtattccatggtgtatatgtaccacattttctttatccagtctatctttgatgggcatttgctattgtgtctttgctattgtgaagagtgctgcaatgaacaaaaatgtgcatgtatctttataataaaatggtttatattcctttgggtatatacccagtaatgggattgctgggacaaatagtatttctagttctagatctttgaggaatagccacacacacttccacaacggttgaactaatttacattcccaccaacaatgtaaaagtgttcctacttctccacagcctcgccagcatctgttgttttttgactttttaataatcaccattctgaccggcatgagatggtatctcattgtggttctcctttgcatttctctaatgatcagtaaggttgagcttttttttatatgtttgttggccacataaatgtcttcttttgagaagtgtctgttcatgtcctttgtccactttttgatggggttgtttttttccttgtaaatttgttttaagttccttgtaggttctggatattagacctttgtcagatggatagattgcaaaaatgttctcccattctgtaggttgcctgttcactctaatgatagtttcttttgctgtgcaggagctctttagtttaattagatcccatttgtaatttttgcttttgttgcaattgcttttgatgtttttgtcatgaaacctttgcttgtgcctatgtcttgaatggtattaaatagattttcttctagggtttttatagttttaggttttacattaagtctttaatcttgagttaatttttgtataaggtgtaaggaaggggtcagtttcaattttctgcatatggctagccagttttcccagcaccatttattaaatagggaatcttttccccattgcttgtttttgtcaggtttgtcgatgatcagatggctgtagatgtgtggtcttctttctctggtctctattctgttccattggtctatgtgtctgtttttgtaccagtaccatgccattttggctactgtagccttgcagtatactttgaagttgggtagtgtgatgcttccagctttgttctttttgcttattgttgtcttggttatacgggctcttttttggttccatttgaattttaaagtagtttttttctaattctgtgaagaatgtcaatagtagtttaatgggaatagcaatgaacctataaattactttgggtagtatggccattttcatgatattgattcttcctatccacgagaatggaatgttttttcatttgtgtcctctcttatttccttgagcagtggtttgtagttctccttgaagagatccttcacatcttattagctgtattcctaggtattttattctctttctagcaactgtgaatgggagttcattcatgatttggctctctgcttgtgtattgttggtgtatagaatgcttgtgatttctgcacattgattttgtatcctgagactttgctgaagttgcttatcagcttaaggaacttttgggtggagataatggggttttctagatatagtatcatgtcatctgcaaacacagttttacttcctcttttcctatttgaataccccttatttgtttctcttgcctgattttcttggccagaacttccaatactatgttaaataggagtggtgagacggcatccctgtcttgtgccagttttcaaggggaatgcttccagcttttgcccattcagtatgataatggctgtgggtttgtcataaatggttattattttgagatattttccatcaatacctagtttattgagagtttttaacatgaagcaacgttgaattttattgaaggccttttctgtatctattgagataatcatgtggtttttgtctttagttctgtttatgtgatgaattatgtttcttgatttgcgtatgttgaaccagccttgcatcccagggatgaagccaacattccaaacattttatttattatttatttatttatttatttttgagacagagtctcgcactgtcgcccaggctggagtgcagtggcaagatctcagctcgctgcaagctccacctcccaggttcatgccgttctcttgcctcggcctcccaaatagcagggactacaggcgaccgccacaacgcctggctaattttttgtatttttagtagagacggggttttacatgttagccaggatggtcttgatctcctgacctcgtgatccgcccgccttggcctcccaaagggctgggattataggcgtgagccaccgcacccggcctccaaacattttaatctcataacaatgcatcacttgggttaactaggttgagataaatataaactgtcaattttttttcccctcacataaaagtccagaggtaggtaattagggctgacacagtgattccagtgattctgctccttcgtgccctcatccaacaaggcttcttgctgctcactacccagctacccctacgtgtggcccgtatcttcatggttcaagatggcagctagagctgctaggtagttaagatctctctcacacactttccttctgtcataattaacacagggttttagctcatgaggccaagcatacacattacttcccactggcacccctatgtaatattaaatgcaaagataccctcaggagtcctgtgctcaaaacaagtacaaaataactttttgttgttgtttgtggtgctggtggttttatttatttattttttctgaaacagggtctcactctgtctcccatgctgaagtgcagtggtgtgatcacagctcatcacaaccttgacctctctgggctcaggggatccactcacttcagcctcccaagtagctgggactacaggaacacgccaccacgctcagctaaattttgtctttttttgtagagatggagtcttgctatgttgcccaggctggtctcaaactcctgggctcaagtgatcagtccacctcagcctcccaaagtactcagattataggtatgagccaccatggcatcaaaataacttggaaagtaggaataattgcttgttgttcctgaaaactgtctcttcgacacttttcagactctgttacatgatcatgacaaaatatacacaaatagacatacagatacacatcagttaaaacctcaagaaatagaaaaataaataaatcataaaatatttaaaaagtggtattctgacacactgcccagaggtacccctgttcagcaattttaaaaaattttaaaaatagccctctccccctccctctcttctccctctccccacggtctccctctgatgccgagccgaagctggactgtactgctgccatctcggctcactgcagcctccctgcctgattctcccgcctcggcctgccgcgtgcctgccattgcgggcgccgccacgcctgactggttttcgtatttttttggtggagacagggtttcactgtgttggccgggctggtctccagctcctgactgcgagtgatctgccagcctcggcctcccgaggtgccgggattgcgggcagagtctcgtccactcagtgctcaatgttgcccaggctggagtgcagtggtgtgatctcagctggctacggcctccgcctcccagccgcctgccttggccccccagggtgccgagattacagcttctgcccggccgccaccccgtctgggatgaagtgaggagcgtctctgcccggccgcccatcgtctgagatgtggggagcgcctctgccccgcccccccgtctgggatgtgaggagcttctctgcccggccaccccgtctgagaagtgaggagcccctccgcccgcagctgccccgtctgagaagtgaggagcccctccgcccgacagccaccctgtctgggaagtgaggagcgtctccgcccagcagccaccccgtctgagaagtgaggagcccctccgcctggcagccgccccgtccgggagggaggcgtgggggtcagcccccgcccggccagccgccccgtcggggagggaggtggggggtcagcccccgcccggccagctatcccgtccgggagggaggtggggggcgcgtccgcctggccgccccatctgggaagtgaggagcccctctgcccagccgccaccccgtctgggaggtgtacccaacagctcattgagaacaggccatgatgacgatggcggttttgtggaatagaaaagggggaaaggtggggaaaagatagagaaatcagattgttgctgtgtctgtgtagaaagaagtagacatgggagacttcattttgttctgtactaagaaaaattcttctgccttaggatgctgttgatctatgaccttacccccaaccctgtgctctctgaaacatgtgctgtgtccactcagggttaaatggattaagggcagtgcaagatgtgctttgttaaacagatgcttgaaggcagcatgctccttaagagtcatcaccactccctaatctcaagtacccagggacacaaacactgcggaaggccgcagggtcctctgcctaggaaaaccagagacctttgttcacttgtttatctgctgaccttccctccactattgtcctgtgaccctgccaaatcaccctctgtgagaaacacccaagaatgatcaattaaaaaaaaaaaatttaaaaataataataggccaggtgcagtggctcacacctgtaatcccagcactttgggaggccgaggctggtgaatcacctgaggtcaggagttcaagaccacgctggccaacatggtggaaaccctgtctccactaaaaatacaaaaattagccgggtgtggtggcaggagcctgtaatcccagctactcgggaggctgaggcaggagaatcgcttgaacccagaaggcagaggttgcaatgagccaagatgatgccactgcactccagcctgggcagcagaatgaaactctgtctcaataataataataataataataataataataataataataataataagcaactctaatgatatttcaaacaatggtccccttttaggtcacactatcaaatcagagaaagatatacttgactagctgtaaaatgcaatttgaggtctaggtgaatgaacaagtaacctctaaatcataaggctattgttacaaactgaatgtttgtattccccccagaattcaaaggggagacagtatccccaaagtgacagtatcagaaggtggggcctttgggaggtaattaggtgatgagggtagagccctcatgaatggaatttgtgcccttaaagatatacttgagagtttgcatcctctttttctgccatgtgagaacatcaaaagactgacatctggtaagatctggaagcatgccttaccagacaccagatatgctaccacttagatgttggatttcccagcctccggaactgtgagaaataactgctgtttaagtcacctggtctatggtaatttggtatagttgcccaaatggactgtgatggttaatactgagtatcaacttgattgaatagaaggatgcaaagtgttcccgggtacatctgtgagggtgctgccaaaggagatttaacatttgagtcagtggactgggaaaggcagaccatcctcaatctgggtgggcaccatctaatcagctgccagcactgccagaataaaagcaggcaaaacatggaaagactagactggtgtagtcttctggcctccatctttctctcatgctgaatgcttcctgccctcaaacattggactccaagttcttcagctttgggacttgaattggcttccttgcttgcagatgacctattgtgggacctaaccctgtgatcatgtgagtcaatactccttaataaactcccctttttatatacatgtatcctattagttctgtccctctagagaaacatgactaatacattgagtaagatagttcctgtcctttttttttttttttaaagagatgggatcttgctatattgcccaggttggtatgcagtggctattcgtaggcacaatcacagcatgctatgaccctgaactcctgggttcaaaagatcctcccacctcagcctcccaagtaactgggaatacaggtacccacacccacacccagctaatttttgtatttttactagggacagcgtttaccatgttggccaggctggtctcgaactcctgacctgaagtgatctgccctccttggcctcccaaagtgctgggattacaggtgtgagccactacgcccagccttttggtttcttatgtgtaggagaggataagtttctttctcagagtgtgctgcagccagacataatatttctccttggcagaaactctgctgttccaatcatacatgtagccattgagttcaatgtgaagatccaggagtgggcgttttctttcttgtctcagtttctgggagaggcactgcaggtacagggatggtgagctgtgagactgctccagcagggacatgtccgcagtacacaggctccagaagaagtcagcttctcggtgaactgtgcacagccctcgcttctgagccttgaattccacattcttcatcgctggcccatccacctccaagaggctgctgtcctccagctggccctctgacaccacatagttctgaataaaaaacatctttggcttccctgctagataagggcatgaatctcccatgaacatcctcctgatgtgatgcagggggagccctgagtgagtctgatccacaccatacacactctgggagcctcctcggctcaccaggacacacacaaagctgtcgtagtctcggtgctcgggcatacaggcaaattggccaagaatctgggatataccatgcatactgagatgcaagaatttctggacttcatagcccagggaagtgaaggtgtctcgaagaagctctgtctcattgccaatgcaatcgattatcaggcagattcctaggggcttgctcttcatcttgtatctctcttcaggtatgctctgaggcaaaaaagcttctgattcctgaatggatttcttcactggttcttgttgagcgccaagctgttccttaagtctttgttctttacttctcccattatggagcctgaagttatttgaaggatccttgagactcttttggattgctgcttggagaacattcctgtaacttgtccctgctccttgaacagactgcttgtacttctggatttttgtcttcaggtctattctgtggatgttctttaggcatttttctaataaatccagttgatctggggcaaccagatttagtttctccaactcaaccacaaggtccaagaaactcttctccttgcttatcttgcctcggcccatgtaatccttcatgaggaaaattaatgaggacacatcagatttatccaaatcctcaccaatctctgccatcagcactgcccgggcagccgccggctcttcccactggatctccgccgggaccaactcccaccctcgccggacaagctcagacctgctgctccgcaaaaccagaattggaaatgctccagatgggacgaggaacaaggacagaaagtcaaaagcatcaacaggtggcttcgccggagggcgtccgagaacctct

SEQ ID NO: 15271 - RNA, 835 nt, Homo sapiens
  source 1..835: mol_type = other RNA
gctgggattacaggcatgagccactgcgcccagccaagacagcattttagatcattccaaacactgctaggggaattttcgtgaggctgaaagtgaagggtttaccagagtacctgatgaaggcaaaggggaagtgctcttgaatccaactgctcaacttcacctcgtataagtgaaaacagagactgcagaacaagctttggcgcctctggctgctcattagcatttacttcagcagcttcttcatcatcaacagcatatgtgactgcgcttagtactttttcttgcattaaaggtgcaatatctcctgaaaaaagtcctggtggtatcttcttagcagtcccttttttgcttcttggacttctttttccaggaatttttttgtcctttcccaagaaggcctgttcatctctggaggcttcacaaagggtgttttgcaagttctcacctgcagccacctcgcagctcaatgtgcagctttcattattattgagactgtcctgctcagacacttggggctttcccatcgcactgtcactgctggtcagatgctcatgcccgtccccgtcaagctgattttcattttcatctgatgcagaaggcagacaggtcacactcctttccacgctgtcaccaggatgacatccatcttgtggttctatttgcagataatatgtaggagtatcgctgtcatccattagagcatcctttggtgaaccatttaaagttacattaaagaccttccatgtctgggaatcggaggcgcaaggagggctaccgctgggcgccgggtctgtttccagccccactcggcgacatggcggccgacgtgctg

SEQ ID NO: 15272 - RNA, 11020 nt, Homo sapiens
  source 1..11020: mol_type = other RNA
gctgggattacaggcatgagccactgcgcccagccacaaatctgagaactttctatgcaatctgcagaaatttttaagaatataaatatgcttttgtcattttatacccagtctggcccaggtttgcactgccataaattcagttttaatgggaacagaagactccagatcctcttgatgggaagaaatcatgaaattttagatgattgacttggttttcatttgtagaaactgggtatgagttggcttaatgaaaatcctaaaataataaaataagcattagtaataatatccttgttaaatgaacaaagtgaatacgatataaagaatgtgataccagaaagttactttaatattgaccctatatagggaagaataatcaaatatttgcaaaatatgttatttttgttttatatatttaacttctaccctatgccacaactgaagacaggttacaagaacatgtgctactacaaagtaggaaactggcagaagccaataagtatcacttaatattttggtatggaaacttttttttttttgagagagttttgctcttgttgcccaggctggagtataatggcacaatctcgactcattgcaacctccacctcctgggttcaagtgattctgctgcctcagcctccctagtagctgggattacaggcatgcgccaccatgcctggctaattttgtatttttagtagagatggggtttctctgtgttggtcaggctggcctcagactccaacctcaggtgatctgcctgcctcagcctcccaaagtgctgggattacaggcgtgagccaccgtgcccagctggaaactttcatttcttaaaacagatttataaaagtttttgctatatagtgactgttagccagtaaaaacagggaagattgattaatttagaagaaattgaaagaaaatatatttattaatgttgcttttaaatgcaaattatcagattgaggagaattttgagaccattgacatttttctaattatgactaaaatttaatcactatacttaataaacatactctattcaaggtcttgtaataaaattatagggaggaataaaacataattgaccccagcgacatcagcaaaaatgggtggactaggaagctgcaagcttttgtttgcctatcaaaacattaaaaaaaaaaaagaggccgggcgtggtggctcacgcctgtaattccagcactttgggaggccgagatgggcagatcacgaggtcaggagatcgagaccatcctggctaacacagtgaaaccccatctctactgaaagtacacaaaattagctgggcatggtggcgggcacctgtagtcctagctacttgggaggctgaggcaggagaatggtgtgaacctgggaggtggagcttgcagtgagccgagatcgtgccactgcactccagcctgggcaatggagcaagactctgtctcaaaaaaaaaaaaaaaaaaaaaaaagcaactgtctgaacgaaccttgttagagctttggaaaacagtcaaaggtttacagcaaccaaaagaatgcccaatcatctgcagaatggtaggaaaatattgtgactttttagtggctcttgcccgagcctctccctacattgtggcagtcttaaagcagcagaagcccagtcccctcccttgaactggagaaaacatgctagaccttttttgcaaattactgtgtacatttttttctaacctgtctgcggatacttgaaggactgacacaaggtcacatgtttgttttgcctaactggtagggtgggcactgcttacaaaagctgcaaagaaccacaggtgcatggggcaagaggttatgggtgtaaacataaaatagaacaactaaggcccagaggagaatctggggtaagactttgggaaattaagaacagttacatatacaggggggatttaaaatgcgacatgcatgcccagggaaaacacttgcccggaaagttctaagacccaagctttcaccttggtctggtccctaagcccaaaagcaggccaaagtaagtattgaaggattacctgggacaaagctgatttgtaaaatctaggattgctcctagcattcaagggaatttatgtcaaaatagctgaacgtgacataaaaggaagagagacttcagtgatcacacacagaaggaatagtcttttataaaaataatttggaaaactctcaaaacaaatggatgacagcttttaaaaataaaaaaacaatgaaccagaaaaccgtggggaaaggaaagaatctcatacctagagttaccatattataatagtgaatatccaactctcaaggaaaaaaatcacaaaccatacaaaggaacaggaaaataatgcgcattcaaaagatcaaaattaattgaccttgtcctaatgaaggacattaaactagacatatactttaactcaaatatgcccaaagaactaaaggaaaacatgaacaaagaattaaagaaatcaggaaaatgataaatgaacaaaatcagaatatcaacagataggcattataaaaaaattctggcagagaaaagtataataaatgaaattttcactacaggggttcagcagcagatataagcaggtagaagaaagaatcagcaaacttgagatgggatcactgaaagcagaaacaacaaatcaagcctacatagttttaaaagatacatatcacacacaaagaagtgaagaagatatggtgcatttttgaaccacaacaggatgtagttagaaatcagtaacaaaaggaaaattggaaaattcacaaacttgtggaaattaaacaaaacactcaaccaatgggtcaaagaagaaatcacaagggaaattaaaaagagaaaaatgcaacataccaaaatttataggatgcagtgaaagcactgctaaaagggaaatttgtagacataaatgcttacattaaaaaacaaaaaagacctcatgtcaacaacctgactttgcagcttgagggggaaaaacatactaaatccaaagctagcagatggaaggaaataataaagattagaacagatataataaattgaataaagattagaaacactagagaaaaatcagtgaaactacaagttctttaaaagaccataaagttggaaagcctatgcgtagatagactaagaaaaaaaggaagactcaattgctaaaataaatgaaaatgggaacagcactctagattctagaaaaatgaaaagggttatagaagaataccttcgacaatctagatgaaatgctcaaagtcctagaaatgcaaaacgtactactgctgaactatgaaaaaaatttaaaaatctcaatagaactataaccagtaaggtaattgaattagtaatcaaaattctcctggaaaaaaagcactggacctgatggttttcatttgtgaattctaccaaataagaagaaataaccccaatcccttctaacttttcccaaaaattgaagaggaaggacgctgcctaattcattctgatgctgaagccagacaaagatactacaagaaaagattacagaccagttattccttatgatcgctgattcaacaattgtcaatactaggaaactgaatttagcagcatattaaaaggattgtacaccacgaccaaatggaatgaattcctggaatgcaaggattgttcaacatacaaaaatcaatataatatactacattaacagaacgaagcgagaaccagatgatcatctcaattgatgcagacaaagcatttgacaaaatccagcagcctcttgtgattaaaaacactcaacaaatgagggataagaggaaactacctgaacataataaaagccagacatgaaaagcccacggtagacaccatacttagtggtgaaagcttttcctctaagatcaagacaatgctcatttcaccattcctattcaacacagtactaggagttctagcctgagctagaaaaagaaaagacatctaagttggaaagtaagaagtaaaatcctatatgttcacaaatgatatgatctttagacaacccgaaagattccacaccaaaaaaaaaaaataactgttaattcagtaaggtagcaggatacaaagtcaacccacaaaagtcagttgcattcctatacactaacaatgaacaacctgagaaggaaattacaagaacagtcccatttaccatagcgtcaaaaagaataaaatgcacagaaattagcttacccaaggtggtaaatggcttgtacaatgaaaactacaaaacattgcttcaataaagataaaaataaacggaaatacatctcatgttcatggattggaaaatctaatgttaatatgtcagtactactcaaagtgatgtgcagattcactacagtctctatcagaatcctaggatttttttttttttttttgcagaaatagaaaaacccatcctgaatttcatgtggaatctgaagggatcccaaatagccaagtcagtcttgagaaagaagaacaaattggaggacttaaacctgcagagtttaaaacttactataatgctacagtaatcaaaacaatgtgattctggcataaaggcagacggatagaccaatgggatagactggagaacctagaaataaaccctctcatatgtaggtaaatgatttttgacaagggtgccaaggctattccaaggatagttttttcaacaaataatgatgggaaagctggataaccacatggctaactaacaaagttgcaacctcactcatttgcaaaaattaactcaaaatggaccaaagacctaaatgtgagagctaaaaccataaaactcttaggatgtggcagtggtttcttggatatgacaccaaattcacagacaacgaaagaaaaaataggcaaattatacttcattaaaattttgtgcatcaaagaacactatcaacagagtaaaaagattacctatggagtgggaggaaataatatgcagttcacgtacctaataaggattaaacatccagaatacatacaaaactcccaaaatgcaacaacagtgtaaaaacctgatttaaaaaatggcaaaggatttggatagatctccagagaggacatgcagatagccagtgagcacaggaaaaaatgcttagcatcactaaacagtaaggaaatgcaaatcaaaaccacattgagataccacttcatacccactgggatagctcttattaaaattaaaaaaacacacaagtgttggcaaggatgtggagaaattggaactcttattactgatggaaatatagtggtatgcagctgctgtagaaaacagtatggtgattttccaattaaatatagaattgtcatttgattcagcaattgcatttctgggtatatacacaaaataattgaaagcggaggcttgagggtatatttgtataccagtgttcactgcagcattattcaccgtagtcaaaaggtagaaacaacccaaatacccaacagatgaatggatagacaaaatgtgttatatccatacaatggaatattattcagccataaaaaggaaatccttctacatactacatcatggatgaacctttcagacattaagtaaatcacaaaaggacaatactatatgaatccactgatgtgaggtacctagactagtgagattcatagagacaaagtagaacaaagattacgttttgtcacagggagcaggagggaatgggaatttattgtttaaggggcacagagattagtgtgggatcatgaaaaagttccggaggtgcatagtggtgactggtacatacaacgaatgtatttaatgcctttaaactgtaacttcaaaatggttaaaatttaaatcttacgtacattttgccacagtaaatttttaaaccaccaaaaaaaaaaaaaaaaaaaaatatggcctagcttttttttttttttttaaaaagggcagggggtggggtatttagtcacaagacatagaggaactttaagtgtatattgctaagtgaaagaagttagtctgaaaggctacatactacatgatttcaaatatatgacattctggagaaagcaaagttagtaaagactggttgccagaggttcagtgggagagagggaggggtaaatacatggagtagagatttttagggtggtgaaactactgtatacaatactataatagtggatacatgacattatatattggtcaaaatccataaagacatacaacaaaaagaggacccttcatgtaaattacaggcttcagctagcctggatgacagagtgagactttgtctcaaaaagtaaagtaaaaatgtgtcaatattggttaaacaaatataccacactagtgcaagatgttaataataaaggcctggggtggggggaagcataggggaactctatactatctgctcagtttttctgaaaatctaaaacttctaataaagtctattaaaattatgtgagagcttttcattttgtgtactctgtctcaatgtcttaccctcatgtgtttgtgaaatgagtgaatgatgggtgatgaatgaattggtgacactagtgacccactgaattcacagcacttacactgggccagactgtgtagagaagccagcgtgcatcccagccttgacgaggacatagttcagagacaggctgttaggtttggccggtgcatgcccttctgcctaagccatttaccagccccagacctttccactgctccaagactttattttcatacttccttaaagttactattgcttttttttcccccatgtaacttaggtagaaaaaactggagaaactaaattgttctgacctaatcagttcttaatattgcacctaaaaagatagaaactgcattctgaaaaatcatgcactaaaaattacaagggaaataggtttggaactttgtgacctgtgtagtacaataacaatcctaaatttccagttacttgcacctagaattagtcaatcttttgcagtcaaaattttgggtttttgtttcttcctttgagagacagatccttgaaatcagtcacttctagtagaaagcattttcatcaatattgaaagaatgatacagaggtatctatcagtcagcgcttttttctaattgccaggtgaaatgtcttctcagttttttcatcagtacttgcagcttctcagataacagcaggaatgaggtggttttgaagccactaagccagctactccttgcatttaaagggttttcatcctttttcataagatcttcatatatcccttagggtttctctctaggtgtgtgaacatttgcctctggttgcttcagcacatcagctttctagtggtgtttcattttctgcctttgtaaaataaaaacaatgatttggttcactttgacgtttcttcagtgttgttcatgactgtggtgggcactggtactgctcgtctctaccaggttgatatcatactggactgaactggctctctgaaagtggcctttcctgcaaaggaagtagaaggctccaatgataagtgttactaggaccgccaatgccacaaaagcttcaaacaggttacttttagtttggatgctggagcctgggagaaaaacctcttcacaacgagctcctgtatagttttcaacgcacctacaaaatgggctgggaatagtaggtatcacataacaaagccccccattcaggcaaaacgacttgtgactgggaccacagggctcttcgtgatctgttggcatcttaatttgtaaatagtttcattcttggtcaagagagtagggttgaaaaacagtaccaagaaatctcttgattataatttgggtttcccatctaggtccaccacctgatctgtccttggatgaaaatttttcctctaaattgcagaatagagaggaaactggttctcttttatggttcaccactatttcttctgctttaatagaatttgtggccacttcaaatttgatgctggttctttatttttctgattcacttttagtctgttagaaagtaaaaagacaaattttctcctttatgtgaaaataatcgtagaatcataaaaatttagagttagaaaaaaacttagagaacttctagatgaagtaagcacaagtctctctaaattagagactttgatttatttcccttactcatagttacagaatgaactggagctggaactctggaatccagaatgtttttcctactacttaatgattcctcaaacttatttaggcacaactttgtgtacatacgtgaggcagtgaggcaccagcgttgaatttaaagtctctgaatcacactgcccaagtttgaatcttggttccttactagctgtgtgatcttgagcaggctacttaatccctctgtgcctcagtttcttcatctcaaaaggtatcttggtatgagagagaatgccaactacagccacgttagaaacgaacagttatgtctggcaaggaagtgatataccaagcttaaacccacagttccacttctgctttacagctcttatactttcctgttgctactaagctcctttactcacaaaattcctctcattagtcacctgcagtgtactgaagcagcacctgtactatttatagctctaggattcccccaccctctcctgtcaataagaatcacctggggcagttaaaaaaaaaatcacaagtcaaccccctgatattagatttcaaggtgtttgaaaggaggctccagaatccgatttttttttctaatcagctgaatttatgactcacagaatctgattttaagcaagtgttcccaagtgagtcttataagccagttaagttcaagaataatgctccaagtgaaagtgagatctgtggcagatcttcacagttcctctagcctcatcagcctcaagggctaatcctcctccggtgttaggcctcagggtatttgaaaacaagagaaggcccagtttgaagaatgcagaatggcatctcgtccacacttaagttttcaataccctaaaaaatttatcgaagggagattttagtttggggaggtgctgtgaagtaagacatcaccagggggcagcatagagttgacaaattatacatgttttgggatttttgacttcacactacaacatgaaatggttgcacctacaatttccattaactcggattactcagaaaaggacaaaacccagaacacttaagacacacgtaaactttattagcatgtaattttcaatacaatggctattatattataaatacataatataaatatttataaatataaatattttctacaatggctattatactataaatagccattgtagaaaaaaatgttcccttgaagtcgcatgaacccgaattcaaaaaaattttattaggatacaaagattcctggtagaaatttgaagtggtcttcaaatttctctcagcaagtttcaaaatacttgtcgtactctgagagttaattagcgttataactggatgcttctcaatagtttcaatcaaatcttaagtagagttctactaaggtggaaaatggagtggataacaatctgggcaagctatgccaaagctttttctaaagaaagtgtacctagttaaaatgctgtcactgactgtcagaaaactatagctcccctcccgtgcatcctccattaatttttcttaacccatctccactttctctattctagtccacatttcttccgtctagaaatgtagaaaaatcctttggcaacccaggtagcttccacaagtatcatctccaagtgtttcttcctctgaaattccaccattagagattagagatgagtaggaaatgctgaaaggcgaaggaggatctgaagaaattttacatttttttctcagtttgccaaaagtagatactccctgtatagatattcccgtataatccagggaaggtagtccaagaccgtggggcaattccaagaggtggttttgaagtccttcaactctaccattttcattttatccatactaaaaaagctacggcaggaagaaaagacaaaggacattcctgggaggccaactggacctaatcaaataaaaacactttagaagaggtacaagaatcagaaatcaaacctatctgcagagccaaaagccattctgaaactccgtgtcctagaaacaagggtttcccatcttttcaaatattttaagataaaaatcgcaacaccctataggaaaatggctatatttttagcaagaattggtggagaagacaaacgataataagctactatgaatccagaagctgcttaaatggccgtattcacagcagcccttgcaaacattaattagagtagtacccattatgggtgaggactttttttttaaccacagagaatatctgtgggtgcatccagattgctcagtggttccgtttaacccacccggtaactggcaatcatggccctaggacaggcttctccaccggggcgatgctgcctccaaggggcgcaatgttactttttatgcatcaagcacggataacacatacagcacataagcaggtcgacagtgtatctgcggtactgggatttcacggggaaaggagatggggacgtgtaaaaagcctttttaagagtcagataacgaaaaacggaaaaagaggagaaacacggtcctacaagggtcctgagctgaggccatcaaatgaatgtactgacaggtatttttctcccaggcagccaactgagagtcaaggcactctgaccgtgctatgactccggccacacagaaagaggtgttttcccctcggtggcctccaagcgcagcgggcactgcgtgccatccgctccctcaccgggcgccccgcgcggatgaaacggagcaactgggaaagagctctggaaactgcaaagcgctgcgccaaagcgacgggaggttcccattctcagctgtacgaaatcccgcgggggtcctccgcttccccgagcgacgccctcggcctccgcacttgttgcttctgcgccccgcctgcgtccccgtcaaaccca

SEQ ID NO: 15273 - RNA, 11211 nt, Homo sapiens
  source 1..11211: mol_type = other RNA
gctgggattacaggcatgagccactgcgcccagccacaaatctgagaactttctatgcaatctgcagaaatttttaagaatataaatatgcttttgtcattttatacccagtctggcccaggtttgcactgccataaattcagttttaatgggaacagaagactccagatcctcttgatgggaagaaatcatgaaattttagatgattgacttggttttcatttgtagaaactgggtatgagttggcttaatgaaaatcctaaaataataaaataagcattagtaataatatccttgttaaatgaacaaagtgaatacgatataaagaatgtgataccagaaagttactttaatattgaccctatatagggaagaataatcaaatatttgcaaaatatgttatttttgttttatatatttaacttctaccctatgccacaactgaagacaggttacaagaacatgtgctactacaaagtaggaaactggcagaagccaataagtatcacttaatattttggtatggaaacttttttttttttgagagagttttgctcttgttgcccaggctggagtataatggcacaatctcgactcattgcaacctccacctcctgggttcaagtgattctgctgcctcagcctccctagtagctgggattacaggcatgcgccaccatgcctggctaattttgtatttttagtagagatggggtttctctgtgttggtcaggctggcctcagactccaacctcaggtgatctgcctgcctcagcctcccaaagtgctgggattacaggcgtgagccaccgtgcccagctggaaactttcatttcttaaaacagatttataaaagtttttgctatatagtgactgttagccagtaaaaacagggaagattgattaatttagaagaaattgaaagaaaatatatttattaatgttgcttttaaatgcaaattatcagattgaggagaattttgagaccattgacatttttctaattatgactaaaatttaatcactatacttaataaacatactctattcaaggtcttgtaataaaattatagggaggaataaaacataattgaccccagcgacatcagcaaaaatgggtggactaggaagctgcaagcttttgtttgcctatcaaaacattaaaaaaaaaaaagaggccgggcgtggtggctcacgcctgtaattccagcactttgggaggccgagatgggcagatcacgaggtcaggagatcgagaccatcctggctaacacagtgaaaccccatctctactgaaagtacacaaaattagctgggcatggtggcgggcacctgtagtcctagctacttgggaggctgaggcaggagaatggtgtgaacctgggaggtggagcttgcagtgagccgagatcgtgccactgcactccagcctgggcaatggagcaagactctgtctcaaaaaaaaaaaaaaaaaaaaaaaagcaactgtctgaacgaaccttgttagagctttggaaaacagtcaaaggtttacagcaaccaaaagaatgcccaatcatctgcagaatggtaggaaaatattgtgactttttagtggctcttgcccgagcctctccctacattgtggcagtcttaaagcagcagaagcccagtcccctcccttgaactggagaaaacatgctagaccttttttgcaaattactgtgtacatttttttctaacctgtctgcggatacttgaaggactgacacaaggtcacatgtttgttttgcctaactggtagggtgggcactgcttacaaaagctgcaaagaaccacaggtgcatggggcaagaggttatgggtgtaaacataaaatagaacaactaaggcccagaggagaatctggggtaagactttgggaaattaagaacagttacatatacaggggggatttaaaatgcgacatgcatgcccagggaaaacacttgcccggaaagttctaagacccaagctttcaccttggtctggtccctaagcccaaaagcaggccaaagtaagtattgaaggattacctgggacaaagctgatttgtaaaatctaggattgctcctagcattcaagggaatttatgtcaaaatagctgaacgtgacataaaaggaagagagacttcagtgatcacacacagaaggaatagtcttttataaaaataatttggaaaactctcaaaacaaatggatgacagcttttaaaaataaaaaaacaatgaaccagaaaaccgtggggaaaggaaagaatctcatacctagagttaccatattataatagtgaatatccaactctcaaggaaaaaaatcacaaaccatacaaaggaacaggaaaataatgcgcattcaaaagatcaaaattaattgaccttgtcctaatgaaggacattaaactagacatatactttaactcaaatatgcccaaagaactaaaggaaaacatgaacaaagaattaaagaaatcaggaaaatgataaatgaacaaaatcagaatatcaacagataggcattataaaaaaattctggcagagaaaagtataataaatgaaattttcactacaggggttcagcagcagatataagcaggtagaagaaagaatcagcaaacttgagatgggatcactgaaagcagaaacaacaaatcaagcctacatagttttaaaagatacatatcacacacaaagaagtgaagaagatatggtgcatttttgaaccacaacaggatgtagttagaaatcagtaacaaaaggaaaattggaaaattcacaaacttgtggaaattaaacaaaacactcaaccaatgggtcaaagaagaaatcacaagggaaattaaaaagagaaaaatgcaacataccaaaatttataggatgcagtgaaagcactgctaaaagggaaatttgtagacataaatgcttacattaaaaaacaaaaaagacctcatgtcaacaacctgactttgcagcttgagggggaaaaacatactaaatccaaagctagcagatggaaggaaataataaagattagaacagatataataaattgaataaagattagaaacactagagaaaaatcagtgaaactacaagttctttaaaagaccataaagttggaaagcctatgcgtagatagactaagaaaaaaaggaagactcaattgctaaaataaatgaaaatgggaacagcactctagattctagaaaaatgaaaagggttatagaagaataccttcgacaatctagatgaaatgctcaaagtcctagaaatgcaaaacgtactactgctgaactatgaaaaaaatttaaaaatctcaatagaactataaccagtaaggtaattgaattagtaatcaaaattctcctggaaaaaaagcactggacctgatggttttcatttgtgaattctaccaaataagaagaaataaccccaatcccttctaacttttcccaaaaattgaagaggaaggacgctgcctaattcattctgatgctgaagccagacaaagatactacaagaaaagattacagaccagttattccttatgatcgctgattcaacaattgtcaatactaggaaactgaatttagcagcatattaaaaggattgtacaccacgaccaaatggaatgaattcctggaatgcaaggattgttcaacatacaaaaatcaatataatatactacattaacagaacgaagcgagaaccagatgatcatctcaattgatgcagacaaagcatttgacaaaatccagcagcctcttgtgattaaaaacactcaacaaatgagggataagaggaaactacctgaacataataaaagccagacatgaaaagcccacggtagacaccatacttagtggtgaaagcttttcctctaagatcaagacaatgctcatttcaccattcctattcaacacagtactaggagttctagcctgagctagaaaaagaaaagacatctaagttggaaagtaagaagtaaaatcctatatgttcacaaatgatatgatctttagacaacccgaaagattccacaccaaaaaaaaaaaataactgttaattcagtaaggtagcaggatacaaagtcaacccacaaaagtcagttgcattcctatacactaacaatgaacaacctgagaaggaaattacaagaacagtcccatttaccatagcgtcaaaaagaataaaatgcacagaaattagcttacccaaggtggtaaatggcttgtacaatgaaaactacaaaacattgcttcaataaagataaaaataaacggaaatacatctcatgttcatggattggaaaatctaatgttaatatgtcagtactactcaaagtgatgtgcagattcactacagtctctatcagaatcctaggatttttttttttttttttgcagaaatagaaaaacccatcctgaatttcatgtggaatctgaagggatcccaaatagccaagtcagtcttgagaaagaagaacaaattggaggacttaaacctgcagagtttaaaacttactataatgctacagtaatcaaaacaatgtgattctggcataaaggcagacggatagaccaatgggatagactggagaacctagaaataaaccctctcatatgtaggtaaatgatttttgacaagggtgccaaggctattccaaggatagttttttcaacaaataatgatgggaaagctggataaccacatggctaactaacaaagttgcaacctcactcatttgcaaaaattaactcaaaatggaccaaagacctaaatgtgagagctaaaaccataaaactcttaggatgtggcagtggtttcttggatatgacaccaaattcacagacaacgaaagaaaaaataggcaaattatacttcattaaaattttgtgcatcaaagaacactatcaacagagtaaaaagattacctatggagtgggaggaaataatatgcagttcacgtacctaataaggattaaacatccagaatacatacaaaactcccaaaatgcaacaacagtgtaaaaacctgatttaaaaaatggcaaaggatttggatagatctccagagaggacatgcagatagccagtgagcacaggaaaaaatgcttagcatcactaaacagtaaggaaatgcaaatcaaaaccacattgagataccacttcatacccactgggatagctcttattaaaattaaaaaaacacacaagtgttggcaaggatgtggagaaattggaactcttattactgatggaaatatagtggtatgcagctgctgtagaaaacagtatggtgattttccaattaaatatagaattgtcatttgattcagcaattgcatttctgggtatatacacaaaataattgaaagcggaggcttgagggtatatttgtataccagtgttcactgcagcattattcaccgtagtcaaaaggtagaaacaacccaaatacccaacagatgaatggatagacaaaatgtgttatatccatacaatggaatattattcagccataaaaaggaaatccttctacatactacatcatggatgaacctttcagacattaagtaaatcacaaaaggacaatactatatgaatccactgatgtgaggtacctagactagtgagattcatagagacaaagtagaacaaagattacgttttgtcacagggagcaggagggaatgggaatttattgtttaaggggcacagagattagtgtgggatcatgaaaaagttccggaggtgcatagtggtgactggtacatacaacgaatgtatttaatgcctttaaactgtaacttcaaaatggttaaaatttaaatcttacgtacattttgccacagtaaatttttaaaccaccaaaaaaaaaaaaaaaaaaaaatatggcctagcttttttttttttttttaaaaagggcagggggtggggtatttagtcacaagacatagaggaactttaagtgtatattgctaagtgaaagaagttagtctgaaaggctacatactacatgatttcaaatatatgacattctggagaaagcaaagttagtaaagactggttgccagaggttcagtgggagagagggaggggtaaatacatggagtagagatttttagggtggtgaaactactgtatacaatactataatagtggatacatgacattatatattggtcaaaatccataaagacatacaacaaaaagaggacccttcatgtaaattacaggcttcagctagcctggatgacagagtgagactttgtctcaaaaagtaaagtaaaaatgtgtcaatattggttaaacaaatataccacactagtgcaagatgttaataataaaggcctggggtggggggaagcataggggaactctatactatctgctcagtttttctgaaaatctaaaacttctaataaagtctattaaaattatgtgagagcttttcattttgtgtactctgtctcaatgtcttaccctcatgtgtttgtgaaatgagtgaatgatgggtgatgaatgaattggtgacactagtgacccactgaattcacagcacttacactgggccagactgtgtagagaagccagcgtgcatcccagccttgacgaggacatagttcagagacaggctgttaggtttggccggtgcatgcccttctgcctaagccatttaccagccccagacctttccactgctccaagactttattttcatacttccttaaagttactattgcttttttttcccccatgtaacttaggtagaaaaaactggagaaactaaattgttctgacctaatcagttcttaatattgcacctaaaaagatagaaactgcattctgaaaaatcatgcactaaaaattacaagggaaataggtttggaactttgtgacctgtgtagtacaataacaatcctaaatttccagttacttgcacctagaattagtcaatcttttgcagtcaaaattttgggtttttgtttcttcctttgagagacagatccttgaaatcagtcacttctagtagaaagcattttcatcaatattgaaagaatgatacagaggtatctatcagtcagcgcttttttctaattgccaggtgaaatgtcttctcagttttttcatcagtacttgcagcttctcagataacagcaggaatgaggtggttttgaagccactaagccagctactccttgcatttaaagggttttcatcctttttcataagatcttcatatatcccttagggtttctctctaggtgtgtgaacatttgcctctggttgcttcagcacatcagctttctggggagagtcatgttgaaccaatgtgacttcgaattatactggtatcaccccctacttagcagttgccgatggactgatgcacattacagaagcacacacaccttgcagcagaatggattatggttcatgatacgagttacacaagcgttttatttaagaaataaaggattagatttttaattcttttacctagtggtgtttcattttctgcctttgtaaaataaaaacaatgatttggttcactttgacgtttcttcagtgttgttcatgactgtggtgggcactggtactgctcgtctctaccaggttgatatcatactggactgaactggctctctgaaagtggcctttcctgcaaaggaagtagaaggctccaatgataagtgttactaggaccgccaatgccacaaaagcttcaaacaggttacttttagtttggatgctggagcctgggagaaaaacctcttcacaacgagctcctgtatagttttcaacgcacctacaaaatgggctgggaatagtaggtatcacataacaaagccccccattcaggcaaaacgacttgtgactgggaccacagggctcttcgtgatctgttggcatcttaatttgtaaatagtttcattcttggtcaagagagtagggttgaaaaacagtaccaagaaatctcttgattataatttgggtttcccatctaggtccaccacctgatctgtccttggatgaaaatttttcctctaaattgcagaatagagaggaaactggttctcttttatggttcaccactatttcttctgctttaatagaatttgtggccacttcaaatttgatgctggttctttatttttctgattcacttttagtctgttagaaagtaaaaagacaaattttctcctttatgtgaaaataatcgtagaatcataaaaatttagagttagaaaaaaacttagagaacttctagatgaagtaagcacaagtctctctaaattagagactttgatttatttcccttactcatagttacagaatgaactggagctggaactctggaatccagaatgtttttcctactacttaatgattcctcaaacttatttaggcacaactttgtgtacatacgtgaggcagtgaggcaccagcgttgaatttaaagtctctgaatcacactgcccaagtttgaatcttggttccttactagctgtgtgatcttgagcaggctacttaatccctctgtgcctcagtttcttcatctcaaaaggtatcttggtatgagagagaatgccaactacagccacgttagaaacgaacagttatgtctggcaaggaagtgatataccaagcttaaacccacagttccacttctgctttacagctcttatactttcctgttgctactaagctcctttactcacaaaattcctctcattagtcacctgcagtgtactgaagcagcacctgtactatttatagctctaggattcccccaccctctcctgtcaataagaatcacctggggcagttaaaaaaaaaatcacaagtcaaccccctgatattagatttcaaggtgtttgaaaggaggctccagaatccgatttttttttctaatcagctgaatttatgactcacagaatctgattttaagcaagtgttcccaagtgagtcttataagccagttaagttcaagaataatgctccaagtgaaagtgagatctgtggcagatcttcacagttcctctagcctcatcagcctcaagggctaatcctcctccggtgttaggcctcagggtatttgaaaacaagagaaggcccagtttgaagaatgcagaatggcatctcgtccacacttaagttttcaataccctaaaaaatttatcgaagggagattttagtttggggaggtgctgtgaagtaagacatcaccagggggcagcatagagttgacaaattatacatgttttgggatttttgacttcacactacaacatgaaatggttgcacctacaatttccattaactcggattactcagaaaaggacaaaacccagaacacttaagacacacgtaaactttattagcatgtaattttcaatacaatggctattatattataaatacataatataaatatttataaatataaatattttctacaatggctattatactataaatagccattgtagaaaaaaatgttcccttgaagtcgcatgaacccgaattcaaaaaaattttattaggatacaaagattcctggtagaaatttgaagtggtcttcaaatttctctcagcaagtttcaaaatacttgtcgtactctgagagttaattagcgttataactggatgcttctcaatagtttcaatcaaatcttaagtagagttctactaaggtggaaaatggagtggataacaatctgggcaagctatgccaaagctttttctaaagaaagtgtacctagttaaaatgctgtcactgactgtcagaaaactatagctcccctcccgtgcatcctccattaatttttcttaacccatctccactttctctattctagtccacatttcttccgtctagaaatgtagaaaaatcctttggcaacccaggtagcttccacaagtatcatctccaagtgtttcttcctctgaaattccaccattagagattagagatgagtaggaaatgctgaaaggcgaaggaggatctgaagaaattttacatttttttctcagtttgccaaaagtagatactccctgtatagatattcccgtataatccagggaaggtagtccaagaccgtggggcaattccaagaggtggttttgaagtccttcaactctaccattttcattttatccatactaaaaaagctacggcaggaagaaaagacaaaggacattcctgggaggccaactggacctaatcaaataaaaacactttagaagaggtacaagaatcagaaatcaaacctatctgcagagccaaaagccattctgaaactccgtgtcctagaaacaagggtttcccatcttttcaaatattttaagataaaaatcgcaacaccctataggaaaatggctatatttttagcaagaattggtggagaagacaaacgataataagctactatgaatccagaagctgcttaaatggccgtattcacagcagcccttgcaaacattaattagagtagtacccattatgggtgaggactttttttttaaccacagagaatatctgtgggtgcatccagattgctcagtggttccgtttaacccacccggtaactggcaatcatggccctaggacaggcttctccaccggggcgatgctgcctccaaggggcgcaatgttactttttatgcatcaagcacggataacacatacagcacataagcaggtcgacagtgtatctgcggtactgggatttcacggggaaaggagatggggacgtgtaaaaagcctttttaagagtcagataacgaaaaacggaaaaagaggagaaacacggtcctacaagggtcctgagctgaggccatcaaatgaatgtactgacaggtatttttctcccaggcagccaactgagagtcaaggcactctgaccgtgctatgactccggccacacagaaagaggtgttttcccctcggtggcctccaagcgcagcgggcactgcgtgccatccgctccctcaccgggcgccccgcgcggatgaaacggagcaactgggaaagagctctggaaactgcaaagcgctgcgccaaagcgacgggaggttcccattctcagctgtacgaaatcccgcgggggtcctccgcttccccgagcgacgccctcggcctccgcacttgttgcttctgcgccccgcctgcgtccccgtcaaaccc

SEQ ID NO: 15274 - RNA, 10731 nt, Homo sapiens
  source 1..10731: mol_type = other RNA
gctgggattacaggcatgagccactgcgcccagccacaaatctgagaactttctatgcaatctgcagaaatttttaagaatataaatatgcttttgtcattttatacccagtctggcccaggtttgcactgccataaattcagttttaatgggaacagaagactccagatcctcttgatgggaagaaatcatgaaattttagatgattgacttggttttcatttgtagaaactgggtatgagttggcttaatgaaaatcctaaaataataaaataagcattagtaataatatccttgttaaatgaacaaagtgaatacgatataaagaatgtgataccagaaagttactttaatattgaccctatatagggaagaataatcaaatatttgcaaaatatgttatttttgttttatatatttaacttctaccctatgccacaactgaagacaggttacaagaacatgtgctactacaaagtaggaaactggcagaagccaataagtatcacttaatattttggtatggaaacttttttttttttgagagagttttgctcttgttgcccaggctggagtataatggcacaatctcgactcattgcaacctccacctcctgggttcaagtgattctgctgcctcagcctccctagtagctgggattacaggcatgcgccaccatgcctggctaattttgtatttttagtagagatggggtttctctgtgttggtcaggctggcctcagactccaacctcaggtgatctgcctgcctcagcctcccaaagtgctgggattacaggcgtgagccaccgtgcccagctggaaactttcatttcttaaaacagatttataaaagtttttgctatatagtgactgttagccagtaaaaacagggaagattgattaatttagaagaaattgaaagaaaatatatttattaatgttgcttttaaatgcaaattatcagattgaggagaattttgagaccattgacatttttctaattatgactaaaatttaatcactatacttaataaacatactctattcaaggtcttgtaataaaattatagggaggaataaaacataattgaccccagcgacatcagcaaaaatgggtggactaggaagctgcaagcttttgtttgcctatcaaaacattaaaaaaaaaaaagaggccgggcgtggtggctcacgcctgtaattccagcactttgggaggccgagatgggcagatcacgaggtcaggagatcgagaccatcctggctaacacagtgaaaccccatctctactgaaagtacacaaaattagctgggcatggtggcgggcacctgtagtcctagctacttgggaggctgaggcaggagaatggtgtgaacctgggaggtggagcttgcagtgagccgagatcgtgccactgcactccagcctgggcaatggagcaagactctgtctcaaaaaaaaaaaaaaaaaaaaaaaagcaactgtctgaacgaaccttgttagagctttggaaaacagtcaaaggtttacagcaaccaaaagaatgcccaatcatctgcagaatggtaggaaaatattgtgactttttagtggctcttgcccgagcctctccctacattgtggcagtcttaaagcagcagaagcccagtcccctcccttgaactggagaaaacatgctagaccttttttgcaaattactgtgtacatttttttctaacctgtctgcggatacttgaaggactgacacaaggtcacatgtttgttttgcctaactggtagggtgggcactgcttacaaaagctgcaaagaaccacaggtgcatggggcaagaggttatgggtgtaaacataaaatagaacaactaaggcccagaggagaatctggggtaagactttgggaaattaagaacagttacatatacaggggggatttaaaatgcgacatgcatgcccagggaaaacacttgcccggaaagttctaagacccaagctttcaccttggtctggtccctaagcccaaaagcaggccaaagtaagtattgaaggattacctgggacaaagctgatttgtaaaatctaggattgctcctagcattcaagggaatttatgtcaaaatagctgaacgtgacataaaaggaagagagacttcagtgatcacacacagaaggaatagtcttttataaaaataatttggaaaactctcaaaacaaatggatgacagcttttaaaaataaaaaaacaatgaaccagaaaaccgtggggaaaggaaagaatctcatacctagagttaccatattataatagtgaatatccaactctcaaggaaaaaaatcacaaaccatacaaaggaacaggaaaataatgcgcattcaaaagatcaaaattaattgaccttgtcctaatgaaggacattaaactagacatatactttaactcaaatatgcccaaagaactaaaggaaaacatgaacaaagaattaaagaaatcaggaaaatgataaatgaacaaaatcagaatatcaacagataggcattataaaaaaattctggcagagaaaagtataataaatgaaattttcactacaggggttcagcagcagatataagcaggtagaagaaagaatcagcaaacttgagatgggatcactgaaagcagaaacaacaaatcaagcctacatagttttaaaagatacatatcacacacaaagaagtgaagaagatatggtgcatttttgaaccacaacaggatgtagttagaaatcagtaacaaaaggaaaattggaaaattcacaaacttgtggaaattaaacaaaacactcaaccaatgggtcaaagaagaaatcacaagggaaattaaaaagagaaaaatgcaacataccaaaatttataggatgcagtgaaagcactgctaaaagggaaatttgtagacataaatgcttacattaaaaaacaaaaaagacctcatgtcaacaacctgactttgcagcttgagggggaaaaacatactaaatccaaagctagcagatggaaggaaataataaagattagaacagatataataaattgaataaagattagaaacactagagaaaaatcagtgaaactacaagttctttaaaagaccataaagttggaaagcctatgcgtagatagactaagaaaaaaaggaagactcaattgctaaaataaatgaaaatgggaacagcactctagattctagaaaaatgaaaagggttatagaagaataccttcgacaatctagatgaaatgctcaaagtcctagaaatgcaaaacgtactactgctgaactatgaaaaaaatttaaaaatctcaatagaactataaccagtaaggtaattgaattagtaatcaaaattctcctggaaaaaaagcactggacctgatggttttcatttgtgaattctaccaaataagaagaaataaccccaatcccttctaacttttcccaaaaattgaagaggaaggacgctgcctaattcattctgatgctgaagccagacaaagatactacaagaaaagattacagaccagttattccttatgatcgctgattcaacaattgtcaatactaggaaactgaatttagcagcatattaaaaggattgtacaccacgaccaaatggaatgaattcctggaatgcaaggattgttcaacatacaaaaatcaatataatatactacattaacagaacgaagcgagaaccagatgatcatctcaattgatgcagacaaagcatttgacaaaatccagcagcctcttgtgattaaaaacactcaacaaatgagggataagaggaaactacctgaacataataaaagccagacatgaaaagcccacggtagacaccatacttagtggtgaaagcttttcctctaagatcaagacaatgctcatttcaccattcctattcaacacagtactaggagttctagcctgagctagaaaaagaaaagacatctaagttggaaagtaagaagtaaaatcctatatgttcacaaatgatatgatctttagacaacccgaaagattccacaccaaaaaaaaaaaataactgttaattcagtaaggtagcaggatacaaagtcaacccacaaaagtcagttgcattcctatacactaacaatgaacaacctgagaaggaaattacaagaacagtcccatttaccatagcgtcaaaaagaataaaatgcacagaaattagcttacccaaggtggtaaatggcttgtacaatgaaaactacaaaacattgcttcaataaagataaaaataaacggaaatacatctcatgttcatggattggaaaatctaatgttaatatgtcagtactactcaaagtgatgtgcagattcactacagtctctatcagaatcctaggatttttttttttttttttgcagaaatagaaaaacccatcctgaatttcatgtggaatctgaagggatcccaaatagccaagtcagtcttgagaaagaagaacaaattggaggacttaaacctgcagagtttaaaacttactataatgctacagtaatcaaaacaatgtgattctggcataaaggcagacggatagaccaatgggatagactggagaacctagaaataaaccctctcatatgtaggtaaatgatttttgacaagggtgccaaggctattccaaggatagttttttcaacaaataatgatgggaaagctggataaccacatggctaactaacaaagttgcaacctcactcatttgcaaaaattaactcaaaatggaccaaagacctaaatgtgagagctaaaaccataaaactcttaggatgtggcagtggtttcttggatatgacaccaaattcacagacaacgaaagaaaaaataggcaaattatacttcattaaaattttgtgcatcaaagaacactatcaacagagtaaaaagattacctatggagtgggaggaaataatatgcagttcacgtacctaataaggattaaacatccagaatacatacaaaactcccaaaatgcaacaacagtgtaaaaacctgatttaaaaaatggcaaaggatttggatagatctccagagaggacatgcagatagccagtgagcacaggaaaaaatgcttagcatcactaaacagtaaggaaatgcaaatcaaaaccacattgagataccacttcatacccactgggatagctcttattaaaattaaaaaaacacacaagtgttggcaaggatgtggagaaattggaactcttattactgatggaaatatagtggtatgcagctgctgtagaaaacagtatggtgattttccaattaaatatagaattgtcatttgattcagcaattgcatttctgggtatatacacaaaataattgaaagcggaggcttgagggtatatttgtataccagtgttcactgcagcattattcaccgtagtcaaaaggtagaaacaacccaaatacccaacagatgaatggatagacaaaatgtgttatatccatacaatggaatattattcagccataaaaaggaaatccttctacatactacatcatggatgaacctttcagacattaagtaaatcacaaaaggacaatactatatgaatccactgatgtgaggtacctagactagtgagattcatagagacaaagtagaacaaagattacgttttgtcacagggagcaggagggaatgggaatttattgtttaaggggcacagagattagtgtgggatcatgaaaaagttccggaggtgcatagtggtgactggtacatacaacgaatgtatttaatgcctttaaactgtaacttcaaaatggttaaaatttaaatcttacgtacattttgccacagtaaatttttaaaccaccaaaaaaaaaaaaaaaaaaaaatatggcctagcttttttttttttttttaaaaagggcagggggtggggtatttagtcacaagacatagaggaactttaagtgtatattgctaagtgaaagaagttagtctgaaaggctacatactacatgatttcaaatatatgacattctggagaaagcaaagttagtaaagactggttgccagaggttcagtgggagagagggaggggtaaatacatggagtagagatttttagggtggtgaaactactgtatacaatactataatagtggatacatgacattatatattggtcaaaatccataaagacatacaacaaaaagaggacccttcatgtaaattacaggcttcagctagcctggatgacagagtgagactttgtctcaaaaagtaaagtaaaaatgtgtcaatattggttaaacaaatataccacactagtgcaagatgttaataataaaggcctggggtggggggaagcataggggaactctatactatctgctcagtttttctgaaaatctaaaacttctaataaagtctattaaaattatgtgagagcttttcattttgtgtactctgtctcaatgtcttaccctcatgtgtttgtgaaatgagtgaatgatgggtgatgaatgaattggtgacactagtgacccactgaattcacagcacttacactgggccagactgtgtagagaagccagcgtgcatcccagccttgacgaggacatagttcagagacaggctgttaggtttggccggtgcatgcccttctgcctaagccatttaccagccccagacctttccactgctccaagactttattttcatacttccttaaagttactattgcttttttttcccccatgtaacttaggtagaaaaaactggagaaactaaattgttctgacctaatcagttcttaatattgcacctaaaaagatagaaactgcattctgaaaaatcatgcactaaaaattacaagggaaataggtttggaactttgtgacctgtgtagtacaataacaatcctaaatttccagttacttgcacctagaattagtcaatcttttgcagtcaaaattttgggtttttgtttcttcctttgagagacagatccttgaaatcagtcacttctagtagaaagcattttcatcaatattgaaagaatgatacagaggtatctatcagtcagcgcttttttctaattgccaggtgaaatgtcttctcagttttttcatcagtacttgcagcttctcagataacagcaggaatgaggtggttttgaagccactaagccagctactccttgcatttaaagggttttcatcctttttcataagatcttcatatatcccttagggtttctctctaggtgtgtgaacatttgcctctggttgcttcagcacatcagctttctggggagagtcatgttgaaccaatgtgacttcgaattatactggtatcaccccctacttagcagttgccgatggactgatgcacattacagaagcacacacaccttgcagcagaatggattatggttcatgatacgagttacacaagcgttttatttaagaaataaaggattagatttttaattcttttacctagtggtgtttcattttctgcctttgtaaaataaaaacaatgatttggttcactttgacgtttcttcagtgttgttcatgactgtggtgggcactggtactgctcgtctctaccaggttgatatcatactggactgaactggctctctgaaagtggcctttcctgcaaaggaagtagaaggctccaatgataagtgttactaggaccgccaatgccacaaaagcttcaaacaggttacttttagtttggatgctggagcctgggagaaaaacctcttcacaacgagctcctgtatagttttcaacgcacctacaaaatgggctgggaatagtaggtatcacataacaaagccccccattcaggcaaaacgacttgtgactgggaccacagggctcttcgtgatctgttggcatcttaatttgtaaatagtttcattcttggtcaagagagtagggttgaaaaacagtacctgatctgtccttggatgaaaatttttcctctaaattgcagaatagagaggaaactggttctcttttatggttcaccactatttcttctgctttaatagaatttgtggccactcaaaaggtatcttggtatgagagagaatgccaactacagccacgttagaaacgaacagttatgtctggcaaggaagtgatataccaagcttaaacccacagttccacttctgctttacagctcttatactttcctgttgctactaagctcctttactcacaaaattcctctcattagtcacctgcagtgtactgaagcagcacctgtactatttatagctctaggattcccccaccctctcctgtcaataagaatcacctggggcagttaaaaaaaaaatcacaagtcaaccccctgatattagatttcaaggtgtttgaaaggaggctccagaatccgatttttttttctaatcagctgaatttatgactcacagaatctgattttaagcaagtgttcccaagtgagtcttataagccagttaagttcaagaataatgctccaagtgaaagtgagatctgtggcagatcttcacagttcctctagcctcatcagcctcaagggctaatcctcctccggtgttaggcctcagggtatttgaaaacaagagaaggcccagtttgaagaatgcagaatggcatctcgtccacacttaagttttcaataccctaaaaaatttatcgaagggagattttagtttggggaggtgctgtgaagtaagacatcaccagggggcagcatagagttgacaaattatacatgttttgggatttttgacttcacactacaacatgaaatggttgcacctacaatttccattaactcggattactcagaaaaggacaaaacccagaacacttaagacacacgtaaactttattagcatgtaattttcaatacaatggctattatattataaatacataatataaatatttataaatataaatattttctacaatggctattatactataaatagccattgtagaaaaaaatgttcccttgaagtcgcatgaacccgaattcaaaaaaattttattaggatacaaagattcctggtagaaatttgaagtggtcttcaaatttctctcagcaagtttcaaaatacttgtcgtactctgagagttaattagcgttataactggatgcttctcaatagtttcaatcaaatcttaagtagagttctactaaggtggaaaatggagtggataacaatctgggcaagctatgccaaagctttttctaaagaaagtgtacctagttaaaatgctgtcactgactgtcagaaaactatagctcccctcccgtgcatcctccattaatttttcttaacccatctccactttctctattctagtccacatttcttccgtctagaaatgtagaaaaatcctttggcaacccaggtagcttccacaagtatcatctccaagtgtttcttcctctgaaattccaccattagagattagagatgagtaggaaatgctgaaaggcgaaggaggatctgaagaaattttacatttttttctcagtttgccaaaagtagatactccctgtatagatattcccgtataatccagggaaggtagtccaagaccgtggggcaattccaagaggtggttttgaagtccttcaactctaccattttcattttatccatactaaaaaagctacggcaggaagaaaagacaaaggacattcctgggaggccaactggacctaatcaaataaaaacactttagaagaggtacaagaatcagaaatcaaacctatctgcagagccaaaagccattctgaaactccgtgtcctagaaacaagggtttcccatcttttcaaatattttaagataaaaatcgcaacaccctataggaaaatggctatatttttagcaagaattggtggagaagacaaacgataataagctactatgaatccagaagctgcttaaatggccgtattcacagcagcccttgcaaacattaattagagtagtacccattatgggtgaggactttttttttaaccacagagaatatctgtgggtgcatccagattgctcagtggttccgtttaacccacccggtaactggcaatcatggccctaggacaggcttctccaccggggcgatgctgcctccaaggggcgcaatgttactttttatgcatcaagcacggataacacatacagcacataagcaggtcgacagtgtatctgcggtactgggatttcacggggaaaggagatggggacgtgtaaaaagcctttttaagagtcagataacgaaaaacggaaaaagaggagaaacacggtcctacaagggtcctgagctgaggccatcaaatgaatgtactgacaggtatttttctcccaggcagccaactgagagtcaaggcactctgaccgtgctatgactccggccacacagaaagaggtgttttcccctcggtggcctccaagcgcagcgggcactgcgtgccatccgctccctcaccgggcgccccgcgcggatgaaacggagcaactgggaaagagctctggaaactgcaaagcgctgcgccaaagcgacgggaggttcccattctcagctgtacgaaatcccgcgggggtcctccgcttccccgagcgacgccctcggcctccgcacttgttgcttctgcgccccgcctgcgtccccgtcaaaccc

SEQ ID NO: 15275 - RNA, 17777 nt, Homo sapiens
  source 1..17777: mol_type = other RNA
gctgggattacaggcatgagccactgcgcccagccacaaatctgagaactttctatgcaatctgcagaaatttttaagaatataaatatgcttttgtcattttatacccagtctggcccaggtttgcactgccataaattcagttttaatgggaacagaagactccagatcctcttgatgggaagaaatcatgaaattttagatgattgacttggttttcatttgtagaaactgggtatgagttggcttaatgaaaatcctaaaataataaaataagcattagtaataatatccttgttaaatgaacaaagtgaatacgatataaagaatgtgataccagaaagttactttaatattgaccctatatagggaagaataatcaaatatttgcaaaatatgttatttttgttttatatatttaacttctaccctatgccacaactgaagacaggttacaagaacatgtgctactacaaagtaggaaactggcagaagccaataagtatcacttaatattttggtatggaaacttttttttttttgagagagttttgctcttgttgcccaggctggagtataatggcacaatctcgactcattgcaacctccacctcctgggttcaagtgattctgctgcctcagcctccctagtagctgggattacaggcatgcgccaccatgcctggctaattttgtatttttagtagagatggggtttctctgtgttggtcaggctggcctcagactccaacctcaggtgatctgcctgcctcagcctcccaaagtgctgggattacaggcgtgagccaccgtgcccagctggaaactttcatttcttaaaacagatttataaaagtttttgctatatagtgactgttagccagtaaaaacagggaagattgattaatttagaagaaattgaaagaaaatatatttattaatgttgcttttaaatgcaaattatcagattgaggagaattttgagaccattgacatttttctaattatgactaaaatttaatcactatacttaataaacatactctattcaaggtcttgtaataaaattatagggaggaataaaacataattgaccccagcgacatcagcaaaaatgggtggactaggaagctgcaagcttttgtttgcctatcaaaacattaaaaaaaaaaaagaggccgggcgtggtggctcacgcctgtaattccagcactttgggaggccgagatgggcagatcacgaggtcaggagatcgagaccatcctggctaacacagtgaaaccccatctctactgaaagtacacaaaattagctgggcatggtggcgggcacctgtagtcctagctacttgggaggctgaggcaggagaatggtgtgaacctgggaggtggagcttgcagtgagccgagatcgtgccactgcactccagcctgggcaatggagcaagactctgtctcaaaaaaaaaaaaaaaaaaaaaaaagcaactgtctgaacgaaccttgttagagctttggaaaacagtcaaaggtttacagcaaccaaaagaatgcccaatcatctgcagaatggtaggaaaatattgtgactttttagtggctcttgcccgagcctctccctacattgtggcagtcttaaagcagcagaagcccagtcccctcccttgaactggagaaaacatgctagaccttttttgcaaattactgtgtacatttttttctaacctgtctgcggatacttgaaggactgacacaaggtcacatgtttgttttgcctaactggtagggtgggcactgcttacaaaagctgcaaagaaccacaggtgcatggggcaagaggttatgggtgtaaacataaaatagaacaactaaggcccagaggagaatctggggtaagactttgggaaattaagaacagttacatatacaggggggatttaaaatgcgacatgcatgcccagggaaaacacttgcccggaaagttctaagacccaagctttcaccttggtctggtccctaagcccaaaagcaggccaaagtaagtattgaaggattacctgggacaaagctgatttgtaaaatctaggattgctcctagcattcaagggaatttatgtcaaaatagctgaacgtgacataaaaggaagagagacttcagtgatcacacacagaaggaatagtcttttataaaaataatttggaaaactctcaaaacaaatggatgacagcttttaaaaataaaaaaacaatgaaccagaaaaccgtggggaaaggaaagaatctcatacctagagttaccatattataatagtgaatatccaactctcaaggaaaaaaatcacaaaccatacaaaggaacaggaaaataatgcgcattcaaaagatcaaaattaattgaccttgtcctaatgaaggacattaaactagacatatactttaactcaaatatgcccaaagaactaaaggaaaacatgaacaaagaattaaagaaatcaggaaaatgataaatgaacaaaatcagaatatcaacagataggcattataaaaaaattctggcagagaaaagtataataaatgaaattttcactacaggggttcagcagcagatataagcaggtagaagaaagaatcagcaaacttgagatgggatcactgaaagcagaaacaacaaatcaagcctacatagttttaaaagatacatatcacacacaaagaagtgaagaagatatggtgcatttttgaaccacaacaggatgtagttagaaatcagtaacaaaaggaaaattggaaaattcacaaacttgtggaaattaaacaaaacactcaaccaatgggtcaaagaagaaatcacaagggaaattaaaaagagaaaaatgcaacataccaaaatttataggatgcagtgaaagcactgctaaaagggaaatttgtagacataaatgcttacattaaaaaacaaaaaagacctcatgtcaacaacctgactttgcagcttgagggggaaaaacatactaaatccaaagctagcagatggaaggaaataataaagattagaacagatataataaattgaataaagattagaaacactagagaaaaatcagtgaaactacaagttctttaaaagaccataaagttggaaagcctatgcgtagatagactaagaaaaaaaggaagactcaattgctaaaataaatgaaaatgggaacagcactctagattctagaaaaatgaaaagggttatagaagaataccttcgacaatctagatgaaatgctcaaagtcctagaaatgcaaaacgtactactgctgaactatgaaaaaaatttaaaaatctcaatagaactataaccagtaaggtaattgaattagtaatcaaaattctcctggaaaaaaagcactggacctgatggttttcatttgtgaattctaccaaataagaagaaataaccccaatcccttctaacttttcccaaaaattgaagaggaaggacgctgcctaattcattctgatgctgaagccagacaaagatactacaagaaaagattacagaccagttattccttatgatcgctgattcaacaattgtcaatactaggaaactgaatttagcagcatattaaaaggattgtacaccacgaccaaatggaatgaattcctggaatgcaaggattgttcaacatacaaaaatcaatataatatactacattaacagaacgaagcgagaaccagatgatcatctcaattgatgcagacaaagcatttgacaaaatccagcagcctcttgtgattaaaaacactcaacaaatgagggataagaggaaactacctgaacataataaaagccagacatgaaaagcccacggtagacaccatacttagtggtgaaagcttttcctctaagatcaagacaatgctcatttcaccattcctattcaacacagtactaggagttctagcctgagctagaaaaagaaaagacatctaagttggaaagtaagaagtaaaatcctatatgttcacaaatgatatgatctttagacaacccgaaagattccacaccaaaaaaaaaaaataactgttaattcagtaaggtagcaggatacaaagtcaacccacaaaagtcagttgcattcctatacactaacaatgaacaacctgagaaggaaattacaagaacagtcccatttaccatagcgtcaaaaagaataaaatgcacagaaattagcttacccaaggtggtaaatggcttgtacaatgaaaactacaaaacattgcttcaataaagataaaaataaacggaaatacatctcatgttcatggattggaaaatctaatgttaatatgtcagtactactcaaagtgatgtgcagattcactacagtctctatcagaatcctaggatttttttttttttttttgcagaaatagaaaaacccatcctgaatttcatgtggaatctgaagggatcccaaatagccaagtcagtcttgagaaagaagaacaaattggaggacttaaacctgcagagtttaaaacttactataatgctacagtaatcaaaacaatgtgattctggcataaaggcagacggatagaccaatgggatagactggagaacctagaaataaaccctctcatatgtaggtaaatgatttttgacaagggtgccaaggctattccaaggatagttttttcaacaaataatgatgggaaagctggataaccacatggctaactaacaaagttgcaacctcactcatttgcaaaaattaactcaaaatggaccaaagacctaaatgtgagagctaaaaccataaaactcttaggatgtggcagtggtttcttggatatgacaccaaattcacagacaacgaaagaaaaaataggcaaattatacttcattaaaattttgtgcatcaaagaacactatcaacagagtaaaaagattacctatggagtgggaggaaataatatgcagttcacgtacctaataaggattaaacatccagaatacatacaaaactcccaaaatgcaacaacagtgtaaaaacctgatttaaaaaatggcaaaggatttggatagatctccagagaggacatgcagatagccagtgagcacaggaaaaaatgcttagcatcactaaacagtaaggaaatgcaaatcaaaaccacattgagataccacttcatacccactgggatagctcttattaaaattaaaaaaacacacaagtgttggcaaggatgtggagaaattggaactcttattactgatggaaatatagtggtatgcagctgctgtagaaaacagtatggtgattttccaattaaatatagaattgtcatttgattcagcaattgcatttctgggtatatacacaaaataattgaaagcggaggcttgagggtatatttgtataccagtgttcactgcagcattattcaccgtagtcaaaaggtagaaacaacccaaatacccaacagatgaatggatagacaaaatgtgttatatccatacaatggaatattattcagccataaaaaggaaatccttctacatactacatcatggatgaacctttcagacattaagtaaatcacaaaaggacaatactatatgaatccactgatgtgaggtacctagactagtgagattcatagagacaaagtagaacaaagattacgttttgtcacagggagcaggagggaatgggaatttattgtttaaggggcacagagattagtgtgggatcatgaaaaagttccggaggtgcatagtggtgactggtacatacaacgaatgtatttaatgcctttaaactgtaacttcaaaatggttaaaatttaaatcttacgtacattttgccacagtaaatttttaaaccaccaaaaaaaaaaaaaaaaaaaaatatggcctagcttttttttttttttttaaaaagggcagggggtggggtatttagtcacaagacatagaggaactttaagtgtatattgctaagtgaaagaagttagtctgaaaggctacatactacatgatttcaaatatatgacattctggagaaagcaaagttagtaaagactggttgccagaggttcagtgggagagagggaggggtaaatacatggagtagagatttttagggtggtgaaactactgtatacaatactataatagtggatacatgacattatatattggtcaaaatccataaagacatacaacaaaaagaggacccttcatgtaaattacaggcttcagctagcctggatgacagagtgagactttgtctcaaaaagtaaagtaaaaatgtgtcaatattggttaaacaaatataccacactagtgcaagatgttaataataaaggcctggggtggggggaagcataggggaactctatactatctgctcagtttttctgaaaatctaaaacttctaataaagtctattaaaattatgtgagagcttttcattttgtgtactctgtctcaatgtcttaccctcatgtgtttgtgaaatgagtgaatgatgggtgatgaatgaattggtgacactagtgacccactgaattcacagcacttacactgggccagactgtgtagagaagccagcgtgcatcccagccttgacgaggacatagttcagagacaggctgttaggtttggccggtgcatgcccttctgcctaagccatttaccagccccagacctttccactgctccaagactttattttcatacttccttaaagttactattgcttttttttcccccatgtaacttaggtagaaaaaactggagaaactaaattgttctgacctaatcagttcttaatattgcacctaaaaagatagaaactgcattctgaaaaatcatgcactaaaaattacaagggaaataggtttggaactttgtgacctgtgtagtacaataacaatcctaaatttccagttacttgcacctagaattagtcaatcttttgcagtcaaaattttgggtttttgtttcttcctttgagagacagatccttgaaatcagtcacttctagtagaaagcattttcatcaatattgaaagaatgatacagaggtatctatcagtcagcgcttttttctaattgccaggtgaaatgtcttctcagttttttcatcagtacttgcagcttctcagataacagcaggaatgaggtggttttgaagccactaagccagctactccttgcatttaaagggttttcatcctttttcataagatcttcatatatcccttagggtttctctctaggtgtgtgaacatttgcctctggttgcttcagcacatcagctttctggggagagtcatgttgaaccaatgtgacttcgaattatactggtatcaccccctacttagcagttgccgatggactgatgcacattacagaagcacacacaccttgcagcagaatggattatggttcatgatacgagttacacaagcgttttatttaagaaataaaggattagatttttaattcttttacctagtggtgtttcattttctgcctttgtaaaataaaaacaatgatttggttcactttgacgtttcttcagtgttgttcatgactgtggtgggcactggtactgctcgtctctaccaggttgatatcatactggactgaactggctctctgaaagtggcctttcctgcaaaggaagtagaaggctccaatgataagtgttactaggaccgccaatgccacaaaagcttcaaacaggttacttttagtttggatgctggagcctgggagaaaaacctcttcacaacgagctcctgtatagttttcaacgcacctacaaaatgggctgggaatagtaggtatcacataacaaagccccccattcaggcaaaacgacttgtgactgggaccacagggctcttcgtgatctgttggcatcttaatttgtaaatagtttcattcttggtcaagagagtagggttgaaaaacagtacctgatctgtccttggatgaaaatttttcctctaaattgcagaatagagaggaaactggttctcttttatggttcaccactatttcttctgctttaatagaatttgtggccacttcatccccctggccgggggagccaggcgagggtgcgtggggcagcccagggcttcagctccagcctggagacctgcttcttgtcacatgcttcttatttatttttgcaaactgccctggttcgggtccagctgcagatgccttacctcccattctttgcctccgtgtgccatcttgcatttattaataaaacatgcaagctggaggggggggttgctgctggggggaatcccattgcagtatggcaagcgggcgcctattttcggttttcagacgtggtatagaggtggaaatcccacaccctgaggatttgtggcttggttggtcgtgaccacttcctagtgggcttcccccgtttgtcgggaggtgccccagcggcagaatgggctgtctggaagggatggtgggtcttcaccgtcaggccagaatccccttcaggggacaggtgcaagctagggcaggcagttccctgcttgctaacttgccagggaggcttaaacctagaaaattgtctcccttgatggccgagaaaagatggccttcaacagaatccctgggacttgcatactcaaactcattacggttttgcatctgaacatgactaaagctagccacctgttggaagtcagaccccatgaaacacccccgtaatctagctcacccatccctgtttcacagtcaccaatactgagctagcaataggcccatatgggttccctctatcctctttaatgctgcttggcttttcttttaaaataagacctacctatgatttgatgccctatatgtgagaggttgaaattatatgatttgtttatattccatacacctatcacatcatatcctaaagactgaatttctcttcagtgcatgtgtttatttccctggcttttcaccttgctttgaacaacagtgggaaaatgggatgtatataactgcttacctcctcccccaaatacctccaccctaaaatattgtgatgaaaagaatagtaagagctagaagcaaaaaatgaaaatggttatcacaagatgttgggatatgatagctgaaccgtaattgcttctaaaatggtcagagtgtcacatctaatcacgagaaggacatgtttcttaaatgttcatatgtaccaggtactgagctaaaactatttgtgtatgagctcatttagtcctcacagcaaacctgctatgtccatgttgaagatgaacaagccaggacttagaaaggttaactaacttgcccaaggtcacacagtcagggacagggtaaggatgcaaactcaagcacatggggatactggaggtggggagccctgagggggcttttcctccaggtgcggctgctccgtgtaccttttcattaaaatcaagcttatgcatgagcatgttggcttgggtctaattttccatttcatagattctgcaccaactttgtggctttccagtaagaaaagcagttgtttcagaatggatcagtatggaattttttgaggtggcactaaacctataaaaagtggggtccaagatgtgcttccatttaattctcacacacaaggagttgagtttaaaaagttgtttccctccagatttaaacccataaaacgtatatgcattaagtagaatgaatcactcccattttccattatcgcatcccaccctaccctccttgctgcccttcacactatcttctggtctcactgccagtcatcagagcaacattgtctatcacacttgcctgtgagtgccttaatgggaggaaggaatccatccgtaccagccgtggctcgtaatccagtctctctatgattgtagcaattatgcattcaaagttcttggaatctctgcattcagctatggatgtgtatttaatcatttttttaaagtgcattattataatgcaggtattggattttgttaaacattcctagcagttctcatggacttagaaattgctgtagttgcatcagtgaaaattcacccagtggggctaatagcttttctactcaggtcacatagttgagatagtggtgagaaaggtataggtgaatagaaggaattatttggaaagtatatcccatgcaaataacagcttttaattataaattgatgaataatattaagtaggaaatataagactatctcttttaattttataagctctgtttttgccttggtcaatgtgattggttttagagcaacatgatgttacctttttcattacactgttcttttgaaacagtatagcggtttgtacatagtattcttgcctcgtgggaaacactcagtttaggaggagcacattccctggtgtttacagaaatgctgagacaggatctttctgtcttggggatttccagtctatgatcagataaactcaagatgagtcctgatgttactgggcaagaagcagaaagcaagaggtgttacttgatttctggggaggaaatgagttttcctgtggggagcatcactatcttcttcagttgggaatctcatgattgaagagtttgagaaacggactagtctgctgtcttccattcaagcaggatttcatttaatgcagagctgagaaggctttatcgtgcaaaggccaattcaggaaatataaaagtgtttctggactactttttttttctcttaaaacatatatttaaactgggaaagtcatatgggaaactattaatgcttaagcattatttgtttttattcccttcacgagagtttttgggagagtgggggaaaagttttccaagctatgaaactcacatgtctgtggtgactgattataatgaatattttagtacattgttgaataaggcactaaaactgggatatttgtttttccttgatcgaccttgtaagctacttcattatgaaatgtgttttttcttaaagtatttcttaatttagtattctttaaaatgagatttttattcagttgtcgacagtcttgaatcacaaaagttcacagattactttgaaatacttgattttcatcagtctctgtttcttactatggctgtcgtgtgctgtgtcctgtgataggaagtttcacatctcatattgcagtgaccaccctttgtggtcaactgtttatatgataagaagtgggggagcccaaggtatatgacctaaggggcagagccaagatttgagcccaagtcagcatagctcaaactctgggctcattgccttttgcaccctgactgcaagatgaagcactttctgccccatagttctctggcctcccatcctattctgctccatccacactggcctccttgctgtaccccctgccccaggcccttagcactaatggttctctcccctggaatactcttcccacaggtatcttcatagtccctcgcctcatttcagctttgctcatagtccaaccactcctttaaaactatccccactcccacagcatcctttcctcctccctgtcttgcttttattcgtagcacctcctagcctactatattaattagttgttaagtgtattgcccatctcccccatggaatgaatgctccaaagggcaggggttctgtgtattttgttcactcccccaactctggtactgtgaaaaaagaatcaacaaatcactatggtatccttgaatctttccagcttcccacactttttgtttttgttagtccttactgttctctgtagtgagcaatgaaacctctaaaatgcaaaagctttatgtgttgtttgggggaacagcaagaaagtagagaagaatcgggaaagatctggcttactcttgagccggtgttgggaagagaggaacctgtaaagatggggaaaaagtcacctgagggttgggatgtgtgacgaggcagcaaatggtacgtggggagatggcctgggatggagaagagatctgtgtgggttcccttgtaatgggaatgcataatgtttttgaagaacttccaaaggagactctggattccttcagccatccatcaactctcccagtggcctgagtcactagaaaggaaaaggagcctacggtcattcctactggctttttacacagacaggtgaatccttgcactgcctgcattattagcctgttgcattttttaaacattaaatacctgttggtgtcatccctgtttgagccagggtctgagagttcactgccaaagcacttaccccatgtgtctgagaagcatcacagcctgagatgtctttggtgtaagcagtcccaggaaggactccacatatatctttcattcatctattgtttgcagtagttcttgggccgtagcaaaatcataggcactttgaggactgattcatctgcagaacactttagaatggactacactgggatgctaaagggagttcatggttatggaaagaagcctgggagaaactgctcctcagccacaaaggcctcctctcctcctcccggatggctttaattgctgccctaggcagtctgaattacccgccaggagaggatttccccttcaaaaaacacagcctccctaaaactgcttttgatttgtaatagaaactacttagtagctaggacagaggctgataactcctattcccagaactcattaaaacaaggaattttaataagtatttttgccctttgcagcccaggtttttggaagtccaggcagctgttctctagatttcactgtcaagccgtaatgcatgcaatgcttcagcttctttcccttggctcaaaacaggtctgaagcaagttattttatctacaattccctcacaccatcccaccctggttacacaattgccattttctccagccaatacaatgcataaggccaattaaccttctgcccatgacagtttcctttgaaatagtcaaatctttgtactttacctgaatttgatgcagggcttttaaaaaacaatttctatgacagttactaattctcctttaaccatgactcctaaaatttgttagctttgcccatcaaaacaaaagaacaaggtgaaatatattgcaattcctcaacaaagaaaaagttccattgttttgggacacagtctcaaaagaaaagcttggaaatttctctcccatttctccctgtcttttaactgtcagtttctatgcaaggctctatcactgcccttcttgataccctgcaaggagctcctgcccccacccctctactgaaacagaactcttaaaggtcaccggtgattgcctaatataaatccaatggctgtttctcagatttcgttcatgatggctcagcaacatctgaccccattgacttcctctactctttgaaatgctgtctgtcggcagctccttcctagcggtgtccgtgtctatctggtctctcctctgctgtcatccttcctgttctatcaagaggcagtctgaagtggttaagagtgtgggctctgcctgtgatgtgaatcctggctctagcacttgctagagtagctttgagtaagtgatttaaccctcgtacctcagtgtcctcatcggtaaaatggggagaagagtagctacggcagaggattaaatagtatgcttagtaaagggtaagcacccaacaaatgctatttttttttatcatataacttcctgtgtacatgcctgtaactttagaataaaacccaaatgcctccctctagccatcaggacctctaagatctggctctcgtttagtttgtttatatctcagaccctccccagtgtgcgtccacttctgaggctttgtcccgcgcactccccactcaaccaccctcacctcttcctattctgcccctccttccctggccagaggagggaagaatgccgaggggtgcccctgcccaggagccaccaagcacagcctgctttgtagcagaagacagcctcccttgggcatggagcctgtctctctcagacagagtatgaattacttaagggcaccagctgtgatttatacttttaaaaaatatcttcctcagcatttagcactataactttacacatagtgggaatttaactcatatcttttaactgccaaaacattatggttttacttggcccttccaaaatcctttttcctcctaaattgaaacctgtattgatcagtcctggagctcatgtaagcttgatacgggataattaagtcaacaccacagggagagttacccatgtcagaaccttcttggaacgaggagggatatatagaaataattaaaataatgagagcacagggaataatttaatgcttttaaaaagtagcttgaaatcctaccaacctataaagctgttagaatttttaagaagtgtttagaagttttttctatactctctactctcagaataaaatgagctgtaaagctgtgagtatcaaatctatcaacccttcagaccttgctataggcctgctctggagccactgtgttctagtcctgcttgctttctccttcctgccctggtgaagagggcattgaagttggatgaaaatcaaaggaagggctgcctacttaaaaaaaaaaaaaaaaattaacccctttattggcgttgtgagttggcctggcaaagacagcctaagttttcatcggcatctgctgtgtgtgtccctggggtcatgaagagtgccagagctgtgctgccagtataacagcttcccaccccacaaccctggaagccacaaaggaccatatgctttgcatcttgacattctgtagcagagtttctcaacttcaacactgttgacacatggggccaggtgactctttgttgcaggggcagtcctgtgcattgtaggatatttagcagcatccgtgacccttacccactagatgccaccggtactaccgcgattaccccccgtccccagtggtgacaaccaaaaatgtctccagaaattgccaaatgtcccctagggtgcaaagtcacccccatttgagaaccgttctccataggatcaatacagaaaactcagcatctttctagtttgaagaatacagaacttagataatttgggtcaaatgaagatgaagattgggttataatatacatgaaaggtaaatttgggtttgaaattacacagacaaggaaaatttagactctataagcagttgtagattatatcataaataaggagatgtaaacaaattacagaaatgcagaccatcttcttactcctgaaggcctcgggtctagatgcaacagcacattctgggactgttaaaatcatccttggggctgggtgcggtggttcacgcctataatctcagcactttgggaggccaaggagggcggatcacctaaggtcaggagtttgagaccagcctggccaacatggagaaaccccgtctctactaaaaatacaaaaaattaactggtgtggtggcacatgcctgtactcgggaggctgaggcaggagaatcacttgaaccctggaggcggaggttgcaatgagccgagattgcgccattgcactccagcctgggtgacagagcaaggctgcgtctcaaaaaaaaaaaaaaaaagaaaagaaaagaaaagaaaagaaaaagtcattcttgggtttttttttttttggcattgtatttaagagcttaaagtatgcaataacacatcctgtgactgttaaaatcatccttggggtatttttttgtggggggcattgtaatttaagtgctcaaagtacttgtcggcctttgacaataagtatatcaaaccaaaaataattaatatttctggagaaatctgaaatatttgattatgactggagggaattatatttgacctgcaaagggccagctctccccaccagagcctgcttctgaccataaagccactctaagacagcactcgcaggtgctgcataaagtaggactgacaaggtactttgtgctttgctgaaaggccacaattgctcagtaatcttcatggctcttagaaaatttagctggagacttgtgatttaaaacccacctccaattgacagtcatcattatgttctttctaaatgcagtagcagaaattgcatgccatacccaaaggctaaaagtgacagttaaaatacatgctttctgaaaaactttaaggccccaactttgggagagacctgatttggccagagattacctttggcttgttaattgccctagggatgggaaagtgtttacacagatgatctccaaaatgttccctacgaatagtctagaaataagccttgtgtagtttctcaaaaggaggcaaggtagaattactaattccatagactactgtatcttcagtgttccagacttgtgctaacaggtggaaggaactccaaagatcatatccaatacagtggactgagttgtttcccctccaaaaaatatatgtatatgttgaagccctaacccccaatgtgacttatcaggagatagggtctttaggagataataaaggataaatgatgtcataagggtcggtccctaatctgatagtactgtacccttataaaaagaggaagaaagatactatctctctctcctgcttccatgtgaggacacagtgagaaggtggctgtctgcaagccaggaagagagcccttacagaacttgaccatgctggcatcctgatccaggacttccagccttccagaactgtaagaaaataactttctgttgtttaagccacccaatctatgatattctgttatggcagcctgcactaactaatacatccagcatccttgttgtacagatgaagaaactggatccagacaggtagacttgcaagaggtcaagctactaatgagtggcagggctggaacatagtgcctgtgcttcgtgactcctagcccagtgtacattctccttcccacactttctcccgtcatatggtcatcttatttatcatctctagaacctacagcacatcacttctgtgagcatcagggtccttatgcttgccctgtttatctcaggattgttgcaaggatcagtgacatagcagaaaaaagatagtttaagttttcaaactacaaaatattgtacgaacatgtcatactgaactcagattcggcctagttagcaggaatctatctgcctctggaaattgtaagtctagtcaagtaggtagctctgtgaggtcacactaggctaggtcgactcatgggtgggctggctgttggctttaaggaatagatcaaaggacagaaaaagcaggaggagatagggcctggtttggtgatgaaccacctcaaagcgagatgattgctcttctctttggttgagttgtaaaagctgaggttgatatgagtttgcatagtaagaggaatgttcctcttaaagaggatagactgtcagagctggaggagaccttaagagctcaaggtaccaaccagagtctctggtgttaagcaacagaaacataccctggtgggccgggtgtggtggctcacacctgtaatcccagcattttgggaggccaaggcaggtggatcatctgaggtcaggagttcgagatcagcctggtcaacatggtgaaaccccatctctactaaatacaaaaaattagcgggacatggtggtgcacgcctgtagtcacagctactcgggaggctgaggcaggagaattgcttgaacccgagaggtggactttgcagtgagccaagatcatgccactgcactccagcctgggcagccgagtgaggctctgtctcagaaaagaaaaaa

SEQ ID NO: 15276 - RNA, 1053 nt, Homo sapiens
  source 1..1053: mol_type = other RNA
gctgggattacaggcatgagccactgcgcccagccacaaatctgagaactttctatgcaatctgcagaaatttttaagaatataaatatgcttttgtcattttatacccagtctggcccaggtttgcactgccataaattcagttttaatgggaacagaagactccagatcctcttgatgggaagaaatcatgaaattttagatgattgacttggttttcatttgtagaaactgggtatgagttggcttaatgaaaatcctagtggtgtttcattttctgcctttgtaaaataaaaacaatgatttggttcactttgacgtttcttcagtgttgttcatgaccattttaaccatttttaagttcagtagcattaagtacagtagtcccctcttctccatgggggatacattccaagaccccagtggatgctgtggtgggcactggtactgctcgtctctaccaggttgatatcatactggactgaactggctctctgaaagtggcctttcctgcaaaggaagtagaaggctccaatgataagtgttactaggaccgccaatgccacaaaagcttcaaacaggttacttttagtttggatgctggagcctgggagaaaaacctcttcacaacgagctcctgtatagttttcaacgcacctacaaaatgggctgggaatagtaggtatcacataacaaagccccccattcaggcaaaacgacttgtgactgggaccacagggctcttcgtgatctgttggcatcttaatttgtaaatagtttcattcttggtcaagagagtagggttgaaaaacagtacattatgattacaagctcccagttctgttctataaagaacacttctgacctaaacagaaagactctaacagaaatctcaatctactaacacagttgtaataccaaggtcttctctcaaagccaacagctctttcttagacaagcagagaggcagagaaagcgagcaagcaatcgagagaaacacacacgagcgagaacaggcaggaaggagaacattaaatctatttgatttttaaa

SEQ ID NO: 15277 - RNA, 962 nt, Homo sapiens
  source 1..962: mol_type = other RNA
gctgggattacaggcatgagccactgcgcccagccacaaatctgagaactttctatgcaatctgcagaaatttttaagaatataaatatgcttttgtcattttatacccagtctggcccaggtttgcactgccataaattcagttttaatgggaacagaagactccagatcctcttgatgggaagaaatcatgaaattttagatgattgacttggttttcatttgtagaaactgggtatgagttggcttaatgaaaatcctagtggtgtttcattttctgcctttgtaaaataaaaacaatgatttggttcactttgacgtttcttcagtgttgttcatgaccattttaaccatttttaagttcagtagcattaagtacagtagtcccctcttctccatgggggatacattccaagaccccagtggatgctgtggtgggcactggtactgctcgtctctaccaggttgatatcatactggactgaactggctctctgaaagtggcctttcctgcaaaggaagtagaaggctccaatgataagtgttactaggaccgccaatgccacaaaagcttcaaacaggttacttttagtttggatgctggagcctgggagaaaaacctcttcacaacgagctcctgtatagttttcaacgcacctacaaaatgggctgggaatagtaggtatcacataacaaagccccccattcaggcaaaacgacttgtgactgggaccacagggctcttcgtgatctgttggcatcttaatttgtaaatagtttcattcttggtcaagagagtagggttgaaaaacagtacattcacacaaaaaataaattttgttggacatgcagtgtttcaaaagtttttgaataccgcagacaacagcagctgtgacttgcattttataacatgtcaaaaatctgatttatatggctgcagtgtgcagtgtgggcgaggtcac

SEQ ID NO: 15278 - RNA, 1223 nt, Homo sapiens
  source 1..1223: mol_type = other RNA
gctgggattacaggcatgagccactgcgcccagccacaaatctgagaactttctatgcaatctgcagaaatttttaagaatataaatatgcttttgtcattttatacccagtctggcccaggtttgcactgccataaattcagttttaatgggaacagaagactccagatcctcttgatgggaagaaatcatgaaattttagatgattgacttggttttcatttgtagaaactgggtatgagttggcttaatgaaaatcctagtggtgtttcattttctgcctttgtaaaataaaaacaatgatttggttcactttgacgtttcttcagtgttgttcatgaccattttaaccatttttaagttcagtagcattaagtacagtagtcccctcttctccatgggggatacattccaagaccccagtggatgctgtggtgggcactggtactgctcgtctctaccaggttgatatcatactggactgaactggctctctgaaagtggcctttcctgcaaaggaagtagaaggctccaatgataagtgttactaggaccgccaatgccacaaaagcttcaaacaggttacttttagtttggatgctggagcctgggagaaaaacctcttcacaacgagctcctgtatagttttcaacgcacctacaaaatgggctgggaatagtaggtatcacataacaaagccccccattcaggcaaaacgacttgtgactgggaccacagggctcttcgtgatctgttggcatcttaatttgtaaatagtttcattcttggtcaagagagtagggttgaaaaacagtaccaagaaatctcttgattataatttgggtttcccatctaggtccaccacctgatctgtccttggatgaaaatttttcctctaaattgcagaatagagaggaaactggttctcttttatggttcaccactatttcttctgctttaatagaatttgtggccacttcaaatttgatgctggttctttatttttctgattcacttttagtcgggcgccccgcgcggatgaaacggagcaactgggaaagagctctggaaactgcaaagcgctgcgccaaagcgacgggaggttcccattctcagctgtacgaaatcccgcgggggtcctccgcttccccgagcgacgccctcggcctccgcacttgttgcttctgcgccccgcctgcgtccccgtcaaacccacccttcgc

SEQ ID NO: 15279 - RNA, 3661 nt, Homo sapiens
  source 1..3661: mol_type = other RNA
gctgggattacaggcatgagccactgcgcccagccacaaatctgagaactttctatgcaatctgcagaaatttttaagaatataaatatgcttttgtcattttatacccagtctggcccaggtttgcactgccataaattcagttttaatgggaacagaagactccagatcctcttgatgggaagaaatcatgaaattttagatgattgacttggttttcatttgtagaaactgggtatgagttggcttaatgaaaatcctagtggtgtttcattttctgcctttgtaaaataaaaacaatgatttggttcactttgacgtttcttcagtgttgttcatgaccattttaaccatttttaagttcagtagcattaagtacagtagtcccctcttctccatgggggatacattccaagaccccagtggatgctgtggtgggcactggtactgctcgtctctaccaggttgatatcatactggactgaactggctctctgaaagtggcctttcctgcaaaggaagtagaaggctccaatgataagtgttactaggaccgccaatgccacaaaagcttcaaacaggttacttttagtttggatgctggagcctgggagaaaaacctcttcacaacgagctcctgtatagttttcaacgcacctacaaaatgggctgggaatagtaggtatcacataacaaagccccccattcaggcaaaacgacttgtgactgggaccacagggctcttcgtgatctgttggcatcttaatttgtaaatagtttcattcttggtcaagagagtagggttgaaaaacagtaccaagaaatctcttgattataatttgggtttcccatctaggtccaccacctgatctgtccttggatgaaaatttttcctctaaattgcagaatagagaggaaactggttctcttttatggttcaccactatttcttctgctttaatagaatttgtggccacttcaaatttgatgctggttctttatttttctgattcacttttagtctcaaaaggtatcttggtatgagagagaatgccaactacagccacgttagaaacgaacagttatgtctggcaaggaagtgatataccaagcttaaacccacagttccacttctgctttacagctcttatactttcctgttgctactaagctcctttactcacaaaattcctctcattagtcacctgcagtgtactgaagcagcacctgtactatttatagctctaggattcccccaccctctcctgtcaataagaatcacctggggcagttaaaaaaaaaatcacaagtcaaccccctgatattagatttcaaggtgtttgaaaggaggctccagaatccgatttttttttctaatcagctgaatttatgactcacagaatctgattttaagcaagtgttcccaagtgagtcttataagccagttaagttcaagaataatgctccaagtgaaagtgagatctgtggcagatcttcacagttcctctagcctcatcagcctcaagggctaatcctcctccggtgttaggcctcagggtatttgaaaacaagagaaggcccagtttgaagaatgcagaatggcatctcgtccacacttaagttttcaataccctaaaaaatttatcgaagggagattttagtttggggaggtgctgtgaagtaagacatcaccagggggcagcatagagttgacaaattatacatgttttgggatttttgacttcacactacaacatgaaatggttgcacctacaatttccattaactcggattactcagaaaaggacaaaacccagaacacttaagacacacgtaaactttattagcatgtaattttcaatacaatggctattatattataaatacataatataaatatttataaatataaatattttctacaatggctattatactataaatagccattgtagaaaaaaatgttcccttgaagtcgcatgaacccgaattcaaaaaaattttattaggatacaaagattcctggtagaaatttgaagtggtcttcaaatttctctcagcaagtttcaaaatacttgtcgtactctgagagttaattagcgttataactggatgcttctcaatagtttcaatcaaatcttaagtagagttctactaaggtggaaaatggagtggataacaatctgggcaagctatgccaaagctttttctaaagaaagtgtacctagttaaaatgctgtcactgactgtcagaaaactatagctcccctcccgtgcatcctccattaatttttcttaacccatctccactttctctattctagtccacatttcttccgtctagaaatgtagaaaaatcctttggcaacccaggtagcttccacaagtatcatctccaagtgtttcttcctctgaaattccaccattagagattagagatgagtaggaaatgctgaaaggcgaaggaggatctgaagaaattttacatttttttctcagtttgccaaaagtagatactccctgtatagatattcccgtataatccagggaaggtagtccaagaccgtggggcaattccaagaggtggttttgaagtccttcaactctaccattttcattttatccatactaaaaaagctacggcaggaagaaaagacaaaggacattcctgggaggccaactggacctaatcaaataaaaacactttagaagaggtacaagaatcagaaatcaaacctatctgcagagccaaaagccattctgaaactccgtgtcctagaaacaagggtttcccatcttttcaaatattttaagataaaaatcgcaacaccctataggaaaatggctatatttttagcaagaattggtggagaagacaaacgataataagctactatgaatccagaagctgcttaaatggccgtattcacagcagcccttgcaaacattaattagagtagtacccattatgggtgaggactttttttttaaccacagagaatatctgtgggtgcatccagattgctcagtggttccgtttaacccacccggtaactggcaatcatggccctaggacaggcttctccaccggggcgatgctgcctccaaggggcgcaatgttactttttatgcatcaagcacggataacacatacagcacataagcaggtcgacagtgtatctgcggtactgggatttcacggggaaaggagatggggacgtgtaaaaagcctttttaagagtcagataacgaaaaacggaaaaagaggagaaacacggtcctacaagggtcctgagctgaggccatcaaatgaatgtactgacaggtatttttctcccaggcagccaactgagagtcaaggcactctgaccgtgctatgactccggccacacagaaagaggtgttttcccctcggtggcctccaagcgcagcgggcactgcgtgccatccgctccctcaccgggcgccccgcgcggatgaaacggagcaactgggaaagagctctggaaactgcaaagcgctgcgccaaagcgacgggaggttcccattctcagctgtacgaaatcccgcgggggtcctccgcttccccgagcgacgccctcggcctccgcacttgttgcttctgcgccccgcctgcgtccccgtcaaacccacccttcgc

SEQ ID NO: 15280 - RNA, 1454 nt, Homo sapiens
  source 1..1454: mol_type = other RNA
gctgggattacaggcatgagccactgcgcccagccacaaatctgagaactttctatgcaatctgcagaaatttttaagaatataaatatgcttttgtcattttatacccagtctggcccaggtttgcactgccataaattcagttttaatgggaacagaagactccagatcctcttgatgggaagaaatcatgaaattttagatgattgacttggttttcatttgtagaaactgggtatgagttggcttaatgaaaatcctagtggtgtttcattttctgcctttgtaaaataaaaacaatgatttggttcactttgacgtttcttcagtgttgttcatgaccattttaaccatttttaagttcagtagcattaagtacagtagtcccctcttctccatgggggatacattccaagaccccagtggatgctgtggtgggcactggtactgctcgtctctaccaggttgatatcatactggactgaactggctctctgaaagtggcctttcctgcaaaggaagtagaaggctccaatgataagtgttactaggaccgccaatgccacaaaagcttcaaacaggttacttttagtttggatgctggagcctgggagaaaaacctcttcacaacgagctcctgtatagttttcaacgcacctacaaaatgggctgggaatagtaggtatcacataacaaagccccccattcaggcaaaacgacttgtgactgggaccacagggctcttcgtgatctgttggcatcttaatttgtaaatagtttcattcttggtcaagagagtagggttgaaaaacagtaccaagaaatctcttgattataatttgggtttcccatctaggtccaccacctgatctgtccttggatgaaaatttttcctctaaattgcagaatagagaggaaactggttctcttttatggttcaccactatttcttctgctttaatagaatttgtggccacttcaaatttgatgctggttctttatttttctgattcacttttagtgtgaggcagtgaggcaccagcgttgaatttaaagtctctgaatcacactgcccaagtttgaatcttggttccttactagctgtgtgatcttgagcaggctacttaatccctctgtgcctcagtttcttcatctcaaaaggtatcttggtatgagagagaatgccaactacagccacgttagaaacgaacagttatgtctggcaaggaagtgatataccaagcttaaacccacagttccacttctgctttacagctcttatactttcctgttgctactaagctcctttactcacaaaattcctctcattagtcacctgcagtgtactgaagcagcacctgtactatttatagctctaggattcccccaccctctcctgtcaataagaatcacctggggcagttaaaaaaaaaatcacaagtcaaccccctgat

SEQ ID NO: 15281 - RNA, 980 nt, Homo sapiens
  source 1..980: mol_type = other RNA
gctgggattacaggcatgagccactgcgcccagccacaaatctgagaactttctatgcaatctgcagaaatttttaagaatataaatatgcttttgtcattttatacccagtctggcccaggtttgcactgccataaattcagttttaatgggaacagaagactccagatcctcttgatgggaagaaatcatgaaattttagatgattgacttggttttcatttgtagaaactgggtatgagttggcttaatgaaaatcctagtggtgtttcattttctgcctttgtaaaataaaaacaatgatttggttcactttgacgtttcttcagtgttgttcatgaccattttaaccatttttaagttcagtagcattaagtacagtagtcccctcttctccatgggggatacattccaagaccccagtggatgctgtggtgggcactggtactgctcgtctctaccaggttgatatcatactggactgaactggctctctgaaagtggcctttcctgcaaaggaagtagaaggctccaatgataagtgttactaggaccgccaatgccacaaaagcttcaaacaggttacttttagtttggatgctggagcctgggagaaaaacctcttcacaacgagctcctgtatagttttcaacgcacctacaaaatgggctgggaatagtaggtatcacataacaaagccccccattcaggcaaaacgacttgtgactgggaccacagggctcttcgtgatctgttggcatcttaatttgtaaatagtttcattcttggtcaagagagtagggttgaaaaacagtaccctcaataaaaacttacattcacacaaaaaataaattttgttggacatgcagtgtttcaaaagtttttgaataccgcagacaacagcagctgtgacttgcattttataacatgtcaaaaatctgatttatatggctgcagtgtgcagtgtgggcgaggtcacg

SEQ ID NO: 15282 - RNA, 3999 nt, Homo sapiens
  source 1..3999: mol_type = other RNA
gctgggattacaggcatgagccactgcgcccagccacaaatctgagaactttctatgcaatctgcagaaatttttaagaatataaatatgcttttgtcattttatacccagtctggcccaggtttgcactgccataaattcagttttaatgggaacagaagactccagatcctcttgatgggaagaaatcatgaaattttagatgattgacttggttttcatttgtagaaactgggtatgagttggcttaatgaaaatcctagtggtgtttcattttctgcctttgtaaaataaaaacaatgatttggttcactttgacgtttcttcagtgttgttcatgaccattttaaccatttttaagttcagtagcattaagtacagtagtcccctcttctccatgggggatacattccaagaccccagtggatgctgtggtgggcactggtactgctcgtctctaccaggttgatatcatactggactgaactggctctctgaaagtggcctttcctgcaaaggaagtagaaggctccaatgataagtgttactaggaccgccaatgccacaaaagcttcaaacaggttacttttagtttggatgctggagcctgggagaaaaacctcttcacaacgagctcctgtatagttttcaacgcacctacaaaatgggctgggaatagtaggtatcacataacaaagccccccattcaggcaaaacgacttgtgactgggaccacagggctcttcgtgatctgttggcatcttaatttgtaaatagtttcattcttggtcaagagagtagggttgaaaaacagtacctgatctgtccttggatgaaaatttttcctctaaattgcagaatagagaggaaactggttctcttttatggttcaccactatttcttctgctttaatagaatttgtggccacttcaaatttgatgctggttctttatttttctgattcacttttagtctgttagaaagtaaaaagacaaattttctcctttatgtgaaaataatcgtagaatcataaaaatttagagttagaaaaaaacttagagaacttctagatgaagtaagcacaagtctctctaaattagagactttgatttatttcccttactcatagttacagaatgaactggagctggaactctggaatccagaatgtttttcctactacttaatgattcctcaaacttatttaggcacaactttgtgtacatacgtgaggcagtgaggcaccagcgttgaatttaaagtctctgaatcacactgcccaagtttgaatcttggttccttactagctgtgtgatcttgagcaggctacttaatccctctgtgcctcagtttcttcatctcaaaaggtatcttggtatgagagagaatgccaactacagccacgttagaaacgaacagttatgtctggcaaggaagtgatataccaagcttaaacccacagttccacttctgctttacagctcttatactttcctgttgctactaagctcctttactcacaaaattcctctcattagtcacctgcagtgtactgaagcagcacctgtactatttatagctctaggattcccccaccctctcctgtcaataagaatcacctggggcagttaaaaaaaaaatcacaagtcaaccccctgatattagatttcaaggtgtttgaaaggaggctccagaatccgatttttttttctaatcagctgaatttatgactcacagaatctgattttaagcaagtgttcccaagtgagtcttataagccagttaagttcaagaataatgctccaagtgaaagtgagatctgtggcagatcttcacagttcctctagcctcatcagcctcaagggctaatcctcctccggtgttaggcctcagggtatttgaaaacaagagaaggcccagtttgaagaatgcagaatggcatctcgtccacacttaagttttcaataccctaaaaaatttatcgaagggagattttagtttggggaggtgctgtgaagtaagacatcaccagggggcagcatagagttgacaaattatacatgttttgggatttttgacttcacactacaacatgaaatggttgcacctacaatttccattaactcggattactcagaaaaggacaaaacccagaacacttaagacacacgtaaactttattagcatgtaattttcaatacaatggctattatattataaatacataatataaatatttataaatataaatattttctacaatggctattatactataaatagccattgtagaaaaaaatgttcccttgaagtcgcatgaacccgaattcaaaaaaattttattaggatacaaagattcctggtagaaatttgaagtggtcttcaaatttctctcagcaagtttcaaaatacttgtcgtactctgagagttaattagcgttataactggatgcttctcaatagtttcaatcaaatcttaagtagagttctactaaggtggaaaatggagtggataacaatctgggcaagctatgccaaagctttttctaaagaaagtgtacctagttaaaatgctgtcactgactgtcagaaaactatagctcccctcccgtgcatcctccattaatttttcttaacccatctccactttctctattctagtccacatttcttccgtctagaaatgtagaaaaatcctttggcaacccaggtagcttccacaagtatcatctccaagtgtttcttcctctgaaattccaccattagagattagagatgagtaggaaatgctgaaaggcgaaggaggatctgaagaaattttacatttttttctcagtttgccaaaagtagatactccctgtatagatattcccgtataatccagggaaggtagtccaagaccgtggggcaattccaagaggtggttttgaagtccttcaactctaccattttcattttatccatactaaaaaagctacggcaggaagaaaagacaaaggacattcctgggaggccaactggacctaatcaaataaaaacactttagaagaggtacaagaatcagaaatcaaacctatctgcagagccaaaagccattctgaaactccgtgtcctagaaacaagggtttcccatcttttcaaatattttaagataaaaatcgcaacaccctataggaaaatggctatatttttagcaagaattggtggagaagacaaacgataataagctactatgaatccagaagctgcttaaatggccgtattcacagcagcccttgcaaacattaattagagtagtacccattatgggtgaggactttttttttaaccacagagaatatctgtgggtgcatccagattgctcagtggttccgtttaacccacccggtaactggcaatcatggccctaggacaggcttctccaccggggcgatgctgcctccaaggggcgcaatgttactttttatgcatcaagcacggataacacatacagcacataagcaggtcgacagtgtatctgcggtactgggatttcacggggaaaggagatggggacgtgtaaaaagcctttttaagagtcagataacgaaaaacggaaaaagaggagaaacacggtcctacaagggtcctgagctgaggccatcaaatgaatgtactgacaggtatttttctcccaggcagccaactgagagtcaaggcactctgaccgtgctatgactccggccacacagaaagaggtgttttcccctcggtggcctccaagcgcagcgggcactgcgtgccatccgctccctcaccgggcgccccgcgcggatgaaacggagcaactgggaaagagctctggaaactgcaaagcgctgcgccaaagcgacgggaggttcccattctcagctgtacgaaatcccgcgggggtcctccgcttccccgagcgacgccctcggcctccgcacttgttgcttctgcgccccgcctgcgtccccgtcaaacccacccttcgc

SEQ ID NO: 15283 - RNA, 10604 nt, Homo sapiens
  source 1..10604: mol_type = other RNA
gctgggattacaggcatgagccactgcgcccagccacaaatctgagaactttctatgcaatctgcagaaatttttaagaatataaatatgcttttgtcattttatacccagtctggcccaggtttgcactgccataaattcagttttaatgggaacagaagactccagatcctcttgatgggaagaaatcatgaaattttagatgattgacttggttttcatttgtagaaactgggtatgagttggcttaatgaaaatcctagtggtgtttcattttctgcctttgtaaaataaaaacaatgatttggttcactttgacgtttcttcagtgttgttcatgaccattttaaccatttttaagttcagtagcattaagtacagtagtcccctcttctccatgggggatacattccaagaccccagtggatgctgtggtgggcactggtactgctcgtctctaccaggttgatatcatactggactgaactggctctctgaaagtggcctttcctgcaaaggaagtagaaggctccaatgataagtgttactaggaccgccaatgccacaaaagcttcaaacaggttacttttagtttggatgctggagcctgggagaaaaacctcttcacaacgagctcctgtatagttttcaacgcacctacaaaatgggctgggaatagtaggtatcacataacaaagccccccattcaggcaaaacgacttgtgactgggaccacagggctcttcgtgatctgttggcatcttaatttgtaaatagtttcattcttggtcaagagagtagggttgaaaaacagtacctgatctgtccttggatgaaaatttttcctctaaattgcagaatagagaggaaactggttctcttttatggttcaccactatttcttctgctttaatagaatttgtggccacttcatccccctggccgggggagccaggcgagggtgcgtggggcagcccagggcttcagctccagcctggagacctgcttcttgtcacatgcttcttatttatttttgcaaactgccctggttcgggtccagctgcagatgccttacctcccattctttgcctccgtgtgccatcttgcatttattaataaaacatgcaagctggaggggggggttgctgctggggggaatcccattgcagtatggcaagcgggcgcctattttcggttttcagacgtggtatagaggtggaaatcccacaccctgaggatttgtggcttggttggtcgtgaccacttcctagtgggcttcccccgtttgtcgggaggtgccccagcggcagaatgggctgtctggaagggatggtgggtcttcaccgtcaggccagaatccccttcaggggacaggtgcaagctagggcaggcagttccctgcttgctaacttgccagggaggcttaaacctagaaaattgtctcccttgatggccgagaaaagatggccttcaacagaatccctgggacttgcatactcaaactcattacggttttgcatctgaacatgactaaagctagccacctgttggaagtcagaccccatgaaacacccccgtaatctagctcacccatccctgtttcacagtcaccaatactgagctagcaataggcccatatgggttccctctatcctctttaatgctgcttggcttttcttttaaaataagacctacctatgatttgatgccctatatgtgagaggttgaaattatatgatttgtttatattccatacacctatcacatcatatcctaaagactgaatttctcttcagtgcatgtgtttatttccctggcttttcaccttgctttgaacaacagtgggaaaatgggatgtatataactgcttacctcctcccccaaatacctccaccctaaaatattgtgatgaaaagaatagtaagagctagaagcaaaaaatgaaaatggttatcacaagatgttgggatatgatagctgaaccgtaattgcttctaaaatggtcagagtgtcacatctaatcacgagaaggacatgtttcttaaatgttcatatgtaccaggtactgagctaaaactatttgtgtatgagctcatttagtcctcacagcaaacctgctatgtccatgttgaagatgaacaagccaggacttagaaaggttaactaacttgcccaaggtcacacagtcagggacagggtaaggatgcaaactcaagcacatggggatactggaggtggggagccctgagggggcttttcctccaggtgcggctgctccgtgtaccttttcattaaaatcaagcttatgcatgagcatgttggcttgggtctaattttccatttcatagattctgcaccaactttgtggctttccagtaagaaaagcagttgtttcagaatggatcagtatggaattttttgaggtggcactaaacctataaaaagtggggtccaagatgtgcttccatttaattctcacacacaaggagttgagtttaaaaagttgtttccctccagatttaaacccataaaacgtatatgcattaagtagaatgaatcactcccattttccattatcgcatcccaccctaccctccttgctgcccttcacactatcttctggtctcactgccagtcatcagagcaacattgtctatcacacttgcctgtgagtgccttaatgggaggaaggaatccatccgtaccagccgtggctcgtaatccagtctctctatgattgtagcaattatgcattcaaagttcttggaatctctgcattcagctatggatgtgtatttaatcatttttttaaagtgcattattataatgcaggtattggattttgttaaacattcctagcagttctcatggacttagaaattgctgtagttgcatcagtgaaaattcacccagtggggctaatagcttttctactcaggtcacatagttgagatagtggtgagaaaggtataggtgaatagaaggaattatttggaaagtatatcccatgcaaataacagcttttaattataaattgatgaataatattaagtaggaaatataagactatctcttttaattttataagctctgtttttgccttggtcaatgtgattggttttagagcaacatgatgttacctttttcattacactgttcttttgaaacagtatagcggtttgtacatagtattcttgcctcgtgggaaacactcagtttaggaggagcacattccctggtgtttacagaaatgctgagacaggatctttctgtcttggggatttccagtctatgatcagataaactcaagatgagtcctgatgttactgggcaagaagcagaaagcaagaggtgttacttgatttctggggaggaaatgagttttcctgtggggagcatcactatcttcttcagttgggaatctcatgattgaagagtttgagaaacggactagtctgctgtcttccattcaagcaggatttcatttaatgcagagctgagaaggctttatcgtgcaaaggccaattcaggaaatataaaagtgtttctggactactttttttttctcttaaaacatatatttaaactgggaaagtcatatgggaaactattaatgcttaagcattatttgtttttattcccttcacgagagtttttgggagagtgggggaaaagttttccaagctatgaaactcacatgtctgtggtgactgattataatgaatattttagtacattgttgaataaggcactaaaactgggatatttgtttttccttgatcgaccttgtaagctacttcattatgaaatgtgttttttcttaaagtatttcttaatttagtattctttaaaatgagatttttattcagttgtcgacagtcttgaatcacaaaagttcacagattactttgaaatacttgattttcatcagtctctgtttcttactatggctgtcgtgtgctgtgtcctgtgataggaagtttcacatctcatattgcagtgaccaccctttgtggtcaactgtttatatgataagaagtgggggagcccaaggtatatgacctaaggggcagagccaagatttgagcccaagtcagcatagctcaaactctgggctcattgccttttgcaccctgactgcaagatgaagcactttctgccccatagttctctggcctcccatcctattctgctccatccacactggcctccttgctgtaccccctgccccaggcccttagcactaatggttctctcccctggaatactcttcccacaggtatcttcatagtccctcgcctcatttcagctttgctcatagtccaaccactcctttaaaactatccccactcccacagcatcctttcctcctccctgtcttgcttttattcgtagcacctcctagcctactatattaattagttgttaagtgtattgcccatctcccccatggaatgaatgctccaaagggcaggggttctgtgtattttgttcactcccccaactctggtactgtgaaaaaagaatcaacaaatcactatggtatccttgaatctttccagcttcccacactttttgtttttgttagtccttactgttctctgtagtgagcaatgaaacctctaaaatgcaaaagctttatgtgttgtttgggggaacagcaagaaagtagagaagaatcgggaaagatctggcttactcttgagccggtgttgggaagagaggaacctgtaaagatggggaaaaagtcacctgagggttgggatgtgtgacgaggcagcaaatggtacgtggggagatggcctgggatggagaagagatctgtgtgggttcccttgtaatgggaatgcataatgtttttgaagaacttccaaaggagactctggattccttcagccatccatcaactctcccagtggcctgagtcactagaaaggaaaaggagcctacggtcattcctactggctttttacacagacaggtgaatccttgcactgcctgcattattagcctgttgcattttttaaacattaaatacctgttggtgtcatccctgtttgagccagggtctgagagttcactgccaaagcacttaccccatgtgtctgagaagcatcacagcctgagatgtctttggtgtaagcagtcccaggaaggactccacatatatctttcattcatctattgtttgcagtagttcttgggccgtagcaaaatcataggcactttgaggactgattcatctgcagaacactttagaatggactacactgggatgctaaagggagttcatggttatggaaagaagcctgggagaaactgctcctcagccacaaaggcctcctctcctcctcccggatggctttaattgctgccctaggcagtctgaattacccgccaggagaggatttccccttcaaaaaacacagcctccctaaaactgcttttgatttgtaatagaaactacttagtagctaggacagaggctgataactcctattcccagaactcattaaaacaaggaattttaataagtatttttgccctttgcagcccaggtttttggaagtccaggcagctgttctctagatttcactgtcaagccgtaatgcatgcaatgcttcagcttctttcccttggctcaaaacaggtctgaagcaagttattttatctacaattccctcacaccatcccaccctggttacacaattgccattttctccagccaatacaatgcataaggccaattaaccttctgcccatgacagtttcctttgaaatagtcaaatctttgtactttacctgaatttgatgcagggcttttaaaaaacaatttctatgacagttactaattctcctttaaccatgactcctaaaatttgttagctttgcccatcaaaacaaaagaacaaggtgaaatatattgcaattcctcaacaaagaaaaagttccattgttttgggacacagtctcaaaagaaaagcttggaaatttctctcccatttctccctgtcttttaactgtcagtttctatgcaaggctctatcactgcccttcttgataccctgcaaggagctcctgcccccacccctctactgaaacagaactcttaaaggtcaccggtgattgcctaatataaatccaatggctgtttctcagatttcgttcatgatggctcagcaacatctgaccccattgacttcctctactctttgaaatgctgtctgtcggcagctccttcctagcggtgtccgtgtctatctggtctctcctctgctgtcatccttcctgttctatcaagaggcagtctgaagtggttaagagtgtgggctctgcctgtgatgtgaatcctggctctagcacttgctagagtagctttgagtaagtgatttaaccctcgtacctcagtgtcctcatcggtaaaatggggagaagagtagctacggcagaggattaaatagtatgcttagtaaagggtaagcacccaacaaatgctatttttttttatcatataacttcctgtgtacatgcctgtaactttagaataaaacccaaatgcctccctctagccatcaggacctctaagatctggctctcgtttagtttgtttatatctcagaccctccccagtgtgcgtccacttctgaggctttgtcccgcgcactccccactcaaccaccctcacctcttcctattctgcccctccttccctggccagaggagggaagaatgccgaggggtgcccctgcccaggagccaccaagcacagcctgctttgtagcagaagacagcctcccttgggcatggagcctgtctctctcagacagagtatgaattacttaagggcaccagctgtgatttatacttttaaaaaatatcttcctcagcatttagcactataactttacacatagtgggaatttaactcatatcttttaactgccaaaacattatggttttacttggcccttccaaaatcctttttcctcctaaattgaaacctgtattgatcagtcctggagctcatgtaagcttgatacgggataattaagtcaacaccacagggagagttacccatgtcagaaccttcttggaacgaggagggatatatagaaataattaaaataatgagagcacagggaataatttaatgcttttaaaaagtagcttgaaatcctaccaacctataaagctgttagaatttttaagaagtgtttagaagttttttctatactctctactctcagaataaaatgagctgtaaagctgtgagtatcaaatctatcaacccttcagaccttgctataggcctgctctggagccactgtgttctagtcctgcttgctttctccttcctgccctggtgaagagggcattgaagttggatgaaaatcaaaggaagggctgcctacttaaaaaaaaaaaaaaaaattaacccctttattggcgttgtgagttggcctggcaaagacagcctaagttttcatcggcatctgctgtgtgtgtccctggggtcatgaagagtgccagagctgtgctgccagtataacagcttcccaccccacaaccctggaagccacaaaggaccatatgctttgcatcttgacattctgtagcagagtttctcaacttcaacactgttgacacatggggccaggtgactctttgttgcaggggcagtcctgtgcattgtaggatatttagcagcatccgtgacccttacccactagatgccaccggtactaccgcgattaccccccgtccccagtggtgacaaccaaaaatgtctccagaaattgccaaatgtcccctagggtgcaaagtcacccccatttgagaaccgttctccataggatcaatacagaaaactcagcatctttctagtttgaagaatacagaacttagataatttgggtcaaatgaagatgaagattgggttataatatacatgaaaggtaaatttgggtttgaaattacacagacaaggaaaatttagactctataagcagttgtagattatatcataaataaggagatgtaaacaaattacagaaatgcagaccatcttcttactcctgaaggcctcgggtctagatgcaacagcacattctgggactgttaaaatcatccttggggctgggtgcggtggttcacgcctataatctcagcactttgggaggccaaggagggcggatcacctaaggtcaggagtttgagaccagcctggccaacatggagaaaccccgtctctactaaaaatacaaaaaattaactggtgtggtggcacatgcctgtactcgggaggctgaggcaggagaatcacttgaaccctggaggcggaggttgcaatgagccgagattgcgccattgcactccagcctgggtgacagagcaaggctgcgtctcaaaaaaaaaaaaaaaaagaaaagaaaagaaaagaaaagaaaaagtcattcttgggtttttttttttttggcattgtatttaagagcttaaagtatgcaataacacatcctgtgactgttaaaatcatccttggggtatttttttgtggggggcattgtaatttaagtgctcaaagtacttgtcggcctttgacaataagtatatcaaaccaaaaataattaatatttctggagaaatctgaaatatttgattatgactggagggaattatatttgacctgcaaagggccagctctccccaccagagcctgcttctgaccataaagccactctaagacagcactcgcaggtgctgcataaagtaggactgacaaggtactttgtgctttgctgaaaggccacaattgctcagtaatcttcatggctcttagaaaatttagctggagacttgtgatttaaaacccacctccaattgacagtcatcattatgttctttctaaatgcagtagcagaaattgcatgccatacccaaaggctaaaagtgacagttaaaatacatgctttctgaaaaactttaaggccccaactttgggagagacctgatttggccagagattacctttggcttgttaattgccctagggatgggaaagtgtttacacagatgatctccaaaatgttccctacgaatagtctagaaataagccttgtgtagtttctcaaaaggaggcaaggtagaattactaattccatagactactgtatcttcagtgttccagacttgtgctaacaggtggaaggaactccaaagatcatatccaatacagtggactgagttgtttcccctccaaaaaatatatgtatatgttgaagccctaacccccaatgtgacttatcaggagatagggtctttaggagataataaaggataaatgatgtcataagggtcggtccctaatctgatagtactgtacccttataaaaagaggaagaaagatactatctctctctcctgcttccatgtgaggacacagtgagaaggtggctgtctgcaagccaggaagagagcccttacagaacttgaccatgctggcatcctgatccaggacttccagccttccagaactgtaagaaaataactttctgttgtttaagccacccaatctatgatattctgttatggcagcctgcactaactaatacatccagcatccttgttgtacagatgaagaaactggatccagacaggtagacttgcaagaggtcaagctactaatgagtggcagggctggaacatagtgcctgtgcttcgtgactcctagcccagtgtacattctccttcccacactttctcccgtcatatggtcatcttatttatcatctctagaacctacagcacatcacttctgtgagcatcagggtccttatgcttgccctgtttatctcaggattgttgcaaggatcagtgacatagcagaaaaaagatagtttaagttttcaaactacaaaatattgtacgaacatgtcatactgaactcagattcggcctagttagcaggaatctatctgcctctggaaattgtaagtctagtcaagtaggtagctctgtgaggtcacactaggctaggtcgactcatgggtgggctggctgttggctttaaggaatagatcaaaggacagaaaaagcaggaggagatagggcctggtttggtgatgaaccacctcaaagcgagatgattgctcttctctttggttgagttgtaaaagctgaggttgatatgagtttgcatagtaagaggaatgttcctcttaaagaggatagactgtcagagctggaggagaccttaagagctcaaggtaccaaccagagtctctggtgttaagcaacagaaacataccctggtgggccgggtgtggtggctcacacctgtaatcccagcattttgggaggccaaggcaggtggatcatctgaggtcaggagttcgagatcagcctggtcaacatggtgaaaccccatctctactaaatacaaaaaattagcgggacatggtggtgcacgcctgtagtcacagctactcgggaggctgaggcaggagaattgcttgaacccgagaggtggactttgcagtgagccaagatcatgccactgcactccagcctgggcagccgagtgaggctctgtctcagaaaagaaaaaa

SEQ ID NO: 15284 - RNA, 3950 nt, Homo sapiens
  source 1..3950: mol_type = other RNA
gctgggattacaggcatgagccactgcgcccagccacaaatctgagaactttctatgcaatctgcagaaatttttaagaatataaatatgcttttgtcattttatacccagtctggcccaggtttgcactgccataaattcagttttaatgggaacagaagactccagatcctcttgatgggaagaaatcatgaaattttagatgattgacttggttttcatttgtagaaactgggtatgagttggcttaatgaaaatcctagtggtgtttcattttctgcctttgtaaaataaaaacaatgatttggttcactttgacgtttcttcagtgttgttcatgactgtggtgggcactggtactgctcgtctctaccaggttgatatcatactggactgaactggctctctgaaagtggcctttcctgcaaaggaagtagaaggctccaatgataagtgttactaggaccgccaatgccacaaaagcttcaaacaggttacttttagtttggatgctggagcctgggagaaaaacctcttcacaacgagctcctgtatagttttcaacgcacctacaaaatgggctgggaatagtaggtatcacataacaaagccccccattcaggcaaaacgacttgtgactgggaccacagggctcttcgtgatctgttggcatcttaatttgtaaatagtttcattcttggtcaagagagtagggttgaaaaacagtaccaagaaatctcttgattataatttgggtttcccatctaggtccaccacctgatctgtccttggatgaaaatttttcctctaaattgcagaatagagaggaaactggttctcttttatggttcaccactatttcttctgctttaatagaatttgtggccacttcaaatttgatgctggttctttatttttctgattcacttttagtctgttagaaagtaaaaagacaaattttctcctttatgtgaaaataatcgtagaatcataaaaatttagagttagaaaaaaacttagagaacttctagatgaagtaagcacaagtctctctaaattagagactttgatttatttcccttactcatagttacagaatgaactggagctggaactctggaatccagaatgtttttcctactacttaatgattcctcaaacttatttaggcacaactttgtgtacatacgtgaggcagtgaggcaccagcgttgaatttaaagtctctgaatcacactgcccaagtttgaatcttggttccttactagctgtgtgatcttgagcaggctacttaatccctctgtgcctcagtttcttcatctcaaaaggtatcttggtatgagagagaatgccaactacagccacgttagaaacgaacagttatgtctggcaaggaagtgatataccaagcttaaacccacagttccacttctgctttacagctcttatactttcctgttgctactaagctcctttactcacaaaattcctctcattagtcacctgcagtgtactgaagcagcacctgtactatttatagctctaggattcccccaccctctcctgtcaataagaatcacctggggcagttaaaaaaaaaatcacaagtcaaccccctgatattagatttcaaggtgtttgaaaggaggctccagaatccgatttttttttctaatcagctgaatttatgactcacagaatctgattttaagcaagtgttcccaagtgagtcttataagccagttaagttcaagaataatgctccaagtgaaagtgagatctgtggcagatcttcacagttcctctagcctcatcagcctcaagggctaatcctcctccggtgttaggcctcagggtatttgaaaacaagagaaggcccagtttgaagaatgcagaatggcatctcgtccacacttaagttttcaataccctaaaaaatttatcgaagggagattttagtttggggaggtgctgtgaagtaagacatcaccagggggcagcatagagttgacaaattatacatgttttgggatttttgacttcacactacaacatgaaatggttgcacctacaatttccattaactcggattactcagaaaaggacaaaacccagaacacttaagacacacgtaaactttattagcatgtaattttcaatacaatggctattatattataaatacataatataaatatttataaatataaatattttctacaatggctattatactataaatagccattgtagaaaaaaatgttcccttgaagtcgcatgaacccgaattcaaaaaaattttattaggatacaaagattcctggtagaaatttgaagtggtcttcaaatttctctcagcaagtttcaaaatacttgtcgtactctgagagttaattagcgttataactggatgcttctcaatagtttcaatcaaatcttaagtagagttctactaaggtggaaaatggagtggataacaatctgggcaagctatgccaaagctttttctaaagaaagtgtacctagttaaaatgctgtcactgactgtcagaaaactatagctcccctcccgtgcatcctccattaatttttcttaacccatctccactttctctattctagtccacatttcttccgtctagaaatgtagaaaaatcctttggcaacccaggtagcttccacaagtatcatctccaagtgtttcttcctctgaaattccaccattagagattagagatgagtaggaaatgctgaaaggcgaaggaggatctgaagaaattttacatttttttctcagtttgccaaaagtagatactccctgtatagatattcccgtataatccagggaaggtagtccaagaccgtggggcaattccaagaggtggttttgaagtccttcaactctaccattttcattttatccatactaaaaaagctacggcaggaagaaaagacaaaggacattcctgggaggccaactggacctaatcaaataaaaacactttagaagaggtacaagaatcagaaatcaaacctatctgcagagccaaaagccattctgaaactccgtgtcctagaaacaagggtttcccatcttttcaaatattttaagataaaaatcgcaacaccctataggaaaatggctatatttttagcaagaattggtggagaagacaaacgataataagctactatgaatccagaagctgcttaaatggccgtattcacagcagcccttgcaaacattaattagagtagtacccattatgggtgaggactttttttttaaccacagagaatatctgtgggtgcatccagattgctcagtggttccgtttaacccacccggtaactggcaatcatggccctaggacaggcttctccaccggggcgatgctgcctccaaggggcgcaatgttactttttatgcatcaagcacggataacacatacagcacataagcaggtcgacagtgtatctgcggtactgggatttcacggggaaaggagatggggacgtgtaaaaagcctttttaagagtcagataacgaaaaacggaaaaagaggagaaacacggtcctacaagggtcctgagctgaggccatcaaatgaatgtactgacaggtatttttctcccaggcagccaactgagagtcaaggcactctgaccgtgctatgactccggccacacagaaagaggtgttttcccctcggtggcctccaagcgcagcgggcactgcgtgccatccgctccctcaccgggcgccccgcgcggatgaaacggagcaactgggaaagagctctggaaactgcaaagcgctgcgccaaagcgacgggaggttcccattctcagctgtacgaaatcccgcgggggtcctccgcttccccgagcgacgccctcggcctccgcacttgttgcttctgcgccccgcctgcgtccccgtcaaaccc

SEQ ID NO: 15285 - RNA, 3875 nt, Homo sapiens
  source 1..3875: mol_type = other RNA
gctgggattacaggcatgagccactgcgcccagccacaaatctgagaactttctatgcaatctgcagaaatttttaagaatataaatatgcttttgtcattttatacccagtctggcccaggtttgcactgccataaattcagttttaatgggaacagaagactccagatcctcttgatgggaagaaatcatgaaattttagatgattgacttggttttcatttgtagaaactgggtatgagttggcttaatgaaaatctgtggtgggcactggtactgctcgtctctaccaggttgatatcatactggactgaactggctctctgaaagtggcctttcctgcaaaggaagtagaaggctccaatgataagtgttactaggaccgccaatgccacaaaagcttcaaacaggttacttttagtttggatgctggagcctgggagaaaaacctcttcacaacgagctcctgtatagttttcaacgcacctacaaaatgggctgggaatagtaggtatcacataacaaagccccccattcaggcaaaacgacttgtgactgggaccacagggctcttcgtgatctgttggcatcttaatttgtaaatagtttcattcttggtcaagagagtagggttgaaaaacagtaccaagaaatctcttgattataatttgggtttcccatctaggtccaccacctgatctgtccttggatgaaaatttttcctctaaattgcagaatagagaggaaactggttctcttttatggttcaccactatttcttctgctttaatagaatttgtggccacttcaaatttgatgctggttctttatttttctgattcacttttagtctgttagaaagtaaaaagacaaattttctcctttatgtgaaaataatcgtagaatcataaaaatttagagttagaaaaaaacttagagaacttctagatgaagtaagcacaagtctctctaaattagagactttgatttatttcccttactcatagttacagaatgaactggagctggaactctggaatccagaatgtttttcctactacttaatgattcctcaaacttatttaggcacaactttgtgtacatacgtgaggcagtgaggcaccagcgttgaatttaaagtctctgaatcacactgcccaagtttgaatcttggttccttactagctgtgtgatcttgagcaggctacttaatccctctgtgcctcagtttcttcatctcaaaaggtatcttggtatgagagagaatgccaactacagccacgttagaaacgaacagttatgtctggcaaggaagtgatataccaagcttaaacccacagttccacttctgctttacagctcttatactttcctgttgctactaagctcctttactcacaaaattcctctcattagtcacctgcagtgtactgaagcagcacctgtactatttatagctctaggattcccccaccctctcctgtcaataagaatcacctggggcagttaaaaaaaaaatcacaagtcaaccccctgatattagatttcaaggtgtttgaaaggaggctccagaatccgatttttttttctaatcagctgaatttatgactcacagaatctgattttaagcaagtgttcccaagtgagtcttataagccagttaagttcaagaataatgctccaagtgaaagtgagatctgtggcagatcttcacagttcctctagcctcatcagcctcaagggctaatcctcctccggtgttaggcctcagggtatttgaaaacaagagaaggcccagtttgaagaatgcagaatggcatctcgtccacacttaagttttcaataccctaaaaaatttatcgaagggagattttagtttggggaggtgctgtgaagtaagacatcaccagggggcagcatagagttgacaaattatacatgttttgggatttttgacttcacactacaacatgaaatggttgcacctacaatttccattaactcggattactcagaaaaggacaaaacccagaacacttaagacacacgtaaactttattagcatgtaattttcaatacaatggctattatattataaatacataatataaatatttataaatataaatattttctacaatggctattatactataaatagccattgtagaaaaaaatgttcccttgaagtcgcatgaacccgaattcaaaaaaattttattaggatacaaagattcctggtagaaatttgaagtggtcttcaaatttctctcagcaagtttcaaaatacttgtcgtactctgagagttaattagcgttataactggatgcttctcaatagtttcaatcaaatcttaagtagagttctactaaggtggaaaatggagtggataacaatctgggcaagctatgccaaagctttttctaaagaaagtgtacctagttaaaatgctgtcactgactgtcagaaaactatagctcccctcccgtgcatcctccattaatttttcttaacccatctccactttctctattctagtccacatttcttccgtctagaaatgtagaaaaatcctttggcaacccaggtagcttccacaagtatcatctccaagtgtttcttcctctgaaattccaccattagagattagagatgagtaggaaatgctgaaaggcgaaggaggatctgaagaaattttacatttttttctcagtttgccaaaagtagatactccctgtatagatattcccgtataatccagggaaggtagtccaagaccgtggggcaattccaagaggtggttttgaagtccttcaactctaccattttcattttatccatactaaaaaagctacggcaggaagaaaagacaaaggacattcctgggaggccaactggacctaatcaaataaaaacactttagaagaggtacaagaatcagaaatcaaacctatctgcagagccaaaagccattctgaaactccgtgtcctagaaacaagggtttcccatcttttcaaatattttaagataaaaatcgcaacaccctataggaaaatggctatatttttagcaagaattggtggagaagacaaacgataataagctactatgaatccagaagctgcttaaatggccgtattcacagcagcccttgcaaacattaattagagtagtacccattatgggtgaggactttttttttaaccacagagaatatctgtgggtgcatccagattgctcagtggttccgtttaacccacccggtaactggcaatcatggccctaggacaggcttctccaccggggcgatgctgcctccaaggggcgcaatgttactttttatgcatcaagcacggataacacatacagcacataagcaggtcgacagtgtatctgcggtactgggatttcacggggaaaggagatggggacgtgtaaaaagcctttttaagagtcagataacgaaaaacggaaaaagaggagaaacacggtcctacaagggtcctgagctgaggccatcaaatgaatgtactgacaggtatttttctcccaggcagccaactgagagtcaaggcactctgaccgtgctatgactccggccacacagaaagaggtgttttcccctcggtggcctccaagcgcagcgggcactgcgtgccatccgctccctcaccgggcgccccgcgcggatgaaacggagcaactgggaaagagctctggaaactgcaaagcgctgcgccaaagcgacgggaggttcccattctcagctgtacgaaatcccgcgggggtcctccgcttccccgagcgacgccctcggcctccgcacttgttgcttctgcgccccgcctgcgtccccgtcaaacccacccttcg

SEQ ID NO: 15286 - RNA, 2800 nt, Homo sapiens
  source 1..2800: mol_type = other RNA
gctgggattacaggcatgagccactgcgcccagcccagaacacttttctttgtattttttttatttttatttcttggagacggagtcctgttctgttgcccaggctggagtgctgtggtgagatcttggcttactgcaatctccacctccctggttccagcgattctcctgtcttagcctcccaagtagctgggattacagatgtgcatcaccacgcccagctactttttgtatttttagtagagatgggttttcaccatgttggccaggcgggtcttgaactcctgacctcaggtgatctgcctgcctcggcctcccaaagtgctgggattacaggcgtaagccaccgcgcccagccacagaacattgttaacattcatttttcaggcttttcctaaccatcctatctaaattacgcccttcgtggccctatttttttttttaacaacaaacatctggccttatttattaggcactgttctaaaacctctgcaaggattaacttattcaatcctcaccatagccctctaaggtactcttacttgttctattttagatctacgggggaaattgaggcacagaggggtcagggaacttgcccaggattgtacagctggtgggtggcagagctgggattcaaacccaggcagcttggctttagaatcaacagtctgagcctcatgtcctgctgcccagatctggctgtagacgctctttatttatgtctttctttctctccagctgctgagctgctcaccctttatccactttgcttatcacagtgtctggcacacagtggcattcaagtgctatttgtcaggtgaatgaaggaatgaatgagaaagggggaatttcccataacccaactaccttagcacaataattatggtaattttgacagattgtagatttcaaatcatgggtcaggaaccgctcctgccagtcctgttgtcctgtcatcatctttgaggccagaacagcccagctgtgccaacatacctggggcgagaggcagcccatgttcctcacgccagcggtcagctgcgggttggcctcgggcctgtctctctcttgatctcgcccttactcactccctcgctgtctctctgaacctccttatcgctgtctgcctgtcttgcccacatctccttgttctcattgtgcctctagaccctctttaaagccagtggagtttgaggacatgcaatagtaattttataatcattactgggcagtgtaaaacaaacattagcacagctggcaaagagtgtaggcagatggttcctttgggatcctaaaaaagcaggatacagctgagatctctgtgacactgtggattcagaaactgctggaactgtccagtccctgtggtggctgccccttgtaggggtggtgccaagggtggcttgggggtttaggtcctcctaaatttccattaggccccaacaaatacacaatatagctaaaaaaaaaaaaaacccagtgtatttgttatgaaaatgcaactttgagatgagtctctagaccccacgtcccccctttggataaactctggtgcttcacagctgccggagacccatttgctgtcctctgctttgctaaccatcttcactgagtctttaatatcaagtggggctggaagactgaccagtgccctgattcatttacatattgattcattgcaggtctcaggcacaggttgataattatctaactgtttagattctaacacacattggatggcaatacaaagggcccatgaggcagggtccccttctcaaagaacttcagaggaaaagttaaatggcagtgcaggggttaactgataccatgttggcagcaacagatgttggcagtcagagatgactgtgctgtgtcaaaggcacacaggacaaatatgcacaaccaagctcctaggcaggagagatcctgtgggctgaagagaggtcaggctttgtggaagagtgaatttgccctggggccggaggatgagtaggagctggacagctgagcagggagggtgggggagggtgttccaggctgaggaccagcatggggtgtggctggcagaactagaagtgcagcatgggactatgtgatgagtgggcctagttgggaggtctgacggatatgctcagcccaggcattgagtgtgatgctgatgtcagggctgcccacaaacttaaacaaaagcctgggaacacaaacgtggtatacaccatactaaccaatgtgggaaagaaatcacacatggagccgcttctaagacacattcaataagagcagacatgggtgaccatcctgcgcttctatcctgtgggccagggcagcactcccaggagaaccagcatcttcatgtgccagggtccccttgggaggtgagtctgggcctctcctgtgatgggccagctgcagggtccttccacacgcaggtcctctgctgaaatgacgtggccttggttttgcaggagaacgaggatggtagaataggctggcctgggcaggtgtcccttttagtagtcctctgggtcagtctctctcaaggcctgttgatcctgacagaccccagacaccattcagaaaacacaggaaggcttgttcaccttggaccatcaggctggcattcaagataaaggcaatacccagcgtagtagccatttcatcttcaagtttctgatttgcaactcagaacccctttccctcaagccaccaagctggttccatcctgagaaggaagtcacgaagctgacttctgcgcgcgctcaagcccaggctaaagggggcggggcgaggccgcggg

SEQ ID NO: 15287 - RNA, 2897 nt, Homo sapiens
  source 1..2897: mol_type = other RNA
gctgggattacaggcatgagccactgcgcccagcccagaacacttttctttgtattttttttatttttatttcttggagacggagtcctgttctgttgcccaggctggagtgctgtggtgagatcttggcttactgcaatctccacctccctggttccagcgattctcctgtcttagcctcccaagtagctgggattacagatgtgcatcaccacgcccagctactttttgtatttttagtagagatgggttttcaccatgttggccaggcgggtcttgaactcctgacctcaggtgatctgcctgcctcggcctcccaaagtgctgggattacaggcgtaagccaccgcgcccagccacagaacattgttaacattcatttttcaggcttttcctaaccatcctatctaaattacgcccttcgtggccctatttttttttttaacaacaaacatctggccttatttattaggcactgttctaaaacctctgcaaggattaacttattcaatcctcaccatagccctctaaggtactcttacttgttctattttagatctacgggggaaattgaggcacagaggggtcagggaacttgcccaggattgtacagctggtgggtggcagagctgggattcaaacccaggcagcttggctttagaatcaacagtctgagcctcatgtcctgctgcccagatctggctgtagacgctctttatttatgtctttctttctctccagctgctgagctgctcaccctttatccactttgcttatcacagtgtctggcacacagtggcattcaagtgctatttgtcaggtgaatgaaggaatgaatgagaaagggggaatttcccataacccaactaccttagcacaataattatggtaattttgacagattgtagatttcaaatcatgggtcaggaaccgctcctgccagtcctgttgtcctgtcatcatctttgaggccagaacagcccagctgtgccaacatacctggggcgagaggcagcccatgttcctcacgccagcggtcagctgcgggttggcctcgggcctgtctctctcttgatctcgcccttactcactccctcgctgtctctctgaacctccttatcgctgtctgcctgtcttgcccacatctccttgttctcattgtgcctctagaccctctttaaagccagtggagtttgaggacatgcaatagtaattttataatcattactgggcagtgtaaaacaaacattagcacagctggcaaagagtgtaggcagatggttcctttgggatcctaaaaaagcaggatacagctgagatctctgtgacactgtggattcagaaactgctggaactgtccagtccctgtggtggctgccccttgtaggggtggtgccaagggtggcttgggggtttaggtcctcctaaatttccattaggccccaacaaatacacaatatagctaaaaaaaaaaaaaacccagtgtatttgttatgaaaatgcaactttgagatgagtctctagaccccacgtcccccctttggataaactctggtgcttcacagctgccggagacccatttgctgtcctctgctttgctaaccatcttcactgagtctttaatatcaagtggggctggaagactgaccagtgccctgattcatttacatattgattcattgcaggtctcaggcacaggttgataattatctaactgtttagattctaacacacattggatggcaatacaaagggcccatgaggcagggtccccttctcaaagaacttcagaggaaaagttaaatggcagtgcaggggttaactgataccatgttggcagcaacagatgttggcagtcagagatgactgtgctgtgtcaaaggcacacaggacaaatatgcacaaccaagctcctaggcaggagagatcctgtgggctgaagagaggtcaggctttgtggaagagtgaatttgccctggggccggaggatgagtaggagctggacagctgagcagggagggtgggggagggtgttccaggctgaggaccagcatggggtgtggctggcagaactagaagtgcagcatgggactatgtgatgagtgggcctagttgggaggtctgacggatatgctcagcccaggcattgagtgtgatgctgatgtcagggctgcccacaaacttaaacaaaagcctgggaacacaaacgtggtatacaccatactaaccaatgtgggaaagaaatcacacatggagccgcttctaagacacattcaataagagcagacatgggtgaccatcctgcgcttctatcctgtgggccagggcagcactcccaggagaaccagcatcttcatgtgccagggtccccttgggaggtgagtctgggcctctcctgtgatgggccagctgcagggtccttccacacgcaggtcctctgctgaaatgacgtggccttggttttgcaggagaacgaggatggtagaataggctggcctgggcaggtgtcccttttagtagtcctctgggtcagtctctctcaaggcctgttgatcctgacagaccccagacaccgttccacatggctggggaggccgcacaatcatggtggaaggcaaaggaggcgcaaagacacatcttacatggtggcaggcaaagtgcgggggaacattcagaaaacacaggaaggcttgttcaccttggaccatcaggctggcattcaagataaaggcaatacccagcgtagtagccatttcatcttcaagtttctgatttgcaactcagaacccctttccctcaagccaccaagctggttccatcctgagaaggaagtcacgaagctgacttctgcgcgcgctcaagcccaggctaaagggggcggggcgaggccgcggggg

SEQ ID NO: 15288 - RNA, 1897 nt, Homo sapiens
  source 1..1897: mol_type = other RNA
gctgggattacaggcatgagccactgcgcccagcccccagtgtggttttaattaaagatgggctgctcttgccttgggcttagagtgatgcttagatctttcttctgagttcctgctttgtccctaattttgttcagtccctggacacttggtgcaaaagtagggatcttatctttactcttgatccttccccagcagcaagcttctcttgcttctttctctgggttaggctgctgagtggtggtggtggggatccaattctactgtttggaccactaaaactctgcacctgggatttaaaactaggctttctcagcaacccctactccccagcagcaaacctttgttctgcattagctcagaatgttttggcagataaagttttgtatcttttgctgccaggcaaagcacttttgtttctactttccaccaggacaaatggatcttatctcaatggttatatttgaaaataaaggtatgaattttacattactaaagagaattaaaactaaatttaacagaaattattgcaatatttatatttaagtttcttgaggacacacttaaatattacatttgtaatttgccatgttgacttttaatttataagaactatatcattggattaaagatagtttgaaatgctctgcattcaaattctagtaattccttatgtatatatttctttcttctggatcaaatattcttgtacaaattttaatttttaagtagaaaaaaatatttggagttatgacttaccttcccacacgaaacttttaggtggttatgatgatacaaaatttaccaggtcttctacctgtgcattgcttttatttttctttggataagaaaaaataatgctcactctatcttactggctcatctatctagaatatatgtacacaaacacacagacacttgtattttcttccagaaaccaaattctagaaatttttgaaactataattttcttcttcgtgcactttttttttgccataaacacgtggataagttgtggacattagtaacaaatcaggtatgtcatggcattatgaagtttaaaagtatctgtatgaaataaactctgtacctcattgactcaattcagatatttcttcgttaattaactgaaaagctctacccaaatcatacagccataaagcctctcttttcatctttcaccatcatgaaatactaaatttccttctctactaccagaaatccagtgtttattagtaataaagctaagactcagaagctaaggtatttttccagcaaaccttagggaccctttctctagtattccagatgcacattacaaacagtaggaaaggtaggaagtctttctaaaaaattttccatgtgggatcttgaagacagaattatttactgcccaggctttagttcattgtttcatcattctttttttgaataacatttcataccttatgctttttcttgttttatttttgttatgtgctcagaatggcaaacctgaggtcagaagcagtctatagcttgacagaggatgttttggtcagaagcaggctccagtgtgacagtgggtgtctctggtagcttgagccttatgataatattgcaacacaggaacaactcaaaggtgggaattctgtatctgactttgctcttggacagtcaataccaatcctgcctgttccattttagcaatcagtggaactactctagtcagttgtacaggtggcctcaggtgaaaactcagggcaggacaaatattcaggagatgagacctggtgtatcatggtacatgcactttgcgtcaatctttaaatcttctatttttcaaatggtcgtagttctgaaatgggaatcctgtaaccgtgagcccgcactcctcagcccttgggtggtcgatggg

SEQ ID NO: 15289 - RNA, 2804 nt, Homo sapiens
  source 1..2804: mol_type = other RNA
gctgggattacaggcatgagccactgcgcccagcccctgttcatttttttatgtgtggcccaagacaattcttcttccaatgtagcccagggaagccaaaagattagacgcccctgcttagcatatcctgggtctccctcactcctcgcaatccatcgctgtcccccagggcctccagctgcagcacctctctgtcctgcagccatttacctcatgctcctccctgactgctggactgaggctctgtgaggtcagggcctggcccagacatggctcaatggatgctcaatagaaaggctggatgttggaggtgtgaggacagccagctccactccatcccacagctgtctcctgcagcaacctttctgcaccccctggctcctcctcctgtcattcattcattcaactcatttgttcaactcctgtcatccactcatccaacaaacatagaggacttagcctgtgtcaggctctgactttcagttgggatggaagacagcgtccttacatggacacttggatgactaaggaaggaacttagtaggtgccaaagtgaccctaaggtaggtgcaacctttctgcaccccctggctcctcctcctgtcattcattcattcaactcatttgttcaactcctgtcattcactcatccaacaaacatagaggacttagcctgtgtcaggctctgactttcagttgggatggaagacagcgtccttacatggacacttggatgactaaggaaggaacttagtaggtgccaaagtgaccctaaggtaggtggcctgaggccagcaggtatcctgtgaaaacaatggcagagactcaggctcccatactgggagtcatattattggtgtgcagtacaaaatcactgacaaaacacacctgtgcccatgagccaagcatgcaaagggccaaaggtgtctgctggaatttcttcaaagaggcagctctgtgcgagcactgagcatgcacacttgtggacccctgtcctgggcgaggaccatgcctgagttcttctgctaggagatccaccctctctcccaaatcactcaccagaggttctcccctctgcccaggctcataaagatttgagagctcagccaggtgcggtggctcacgcctgctaatcccagcactttgggaggccgaggcaggcggatcacgaggtcaggagttcgagaccagcctggccaacattgtgaaaccctgtctctactaaaaatacaaaaattagccaggcgtagtggtgcgcacctgtagtcccagctactcaggaggctgaggcaaaagaatcgcttgaaccctggaggcagaggttgcagtgagctgagatcgtgccacggcactccagcctgggcaagagagcgacactccgtctcaaaaaaaaaaacaaaaaaaaaaacacaaagatttgcgagctcagagacaaaggaaatgccatgtgttttccccttcttctgagccccgtggggccagagcacgccttcctctgccttggcaatgacagacaagctggggtccttccccattgccagctctgcagcactgccctcctgggaaccacattcagtcattctgtggagttttcatgatgggtttcatcatcagattcatttcctccatgggagtagactcttcagcaagtcacattacctctccgggcctcagtttcccctcttgtgaaacaacagggtagaacttaagggcccttcctgttttctctgacagtctgaatctgtcttgtgcacgtacatagccctgcaatagtgtcaaagatctttaattgttggatggaaaagaaaggaacctgtgggttttgaggggggacaggtaccgccaaatgcagatgatgattctgagagcacctttgacgggccagatctcgtactctgagtttatctgcgccacttgttgtctggcaagtccagtgatgctgtggtctccagctgattctatctgagctgctcctggggtggcagctctcagaagtgtgggagaggatgcaggcgatggggagggaccgggaccgcatgctccctccaggacatagcgcacaacggtggtctggggtaggatgaagtataagtgctctgcttcaggccagccttgggtgtgagctgtctctgcttgagctgctcatagagtccatagtttgtagggggagcaagaaggggaaagtcagacttctctggcagccacagcaacttctgtccattccaagtgcggagtggaggcagccccgggttgtaaccatgccggttgtaatggtcgtcataggtgctgatcaggtagcgatgtgggggctcctggtggtgggtgatcaggtgtttgtaaggtagcccctcaactttcctcttcccataccacctggagatctggtctggtctgtggtctgggaaggggatgtattcttttctgtaaatggattggggtgtcttgtcagtgtctctggtgaactttctcctctcttccatccaatttccagtgagcactttcgttgaatacttggtctcaatctgccagctcggagtagagagtggctgtggatttactgcagtcaaaaacatgttaaggatttgccccaggtttctttgacttgatgcagtttaaggcttcaggcggggagaggaaggtgttatgaagttgctgagtttggggtgcctattttgtcttcccagctggcctcctgaatggctagtagatgactccttgctaacctcagagaataaaacggccccaagagttcactgtcagcctttagggagagttgatctatcttggattctctactgttgact

SEQ ID NO: 15290 - RNA, 2690 nt, Homo sapiens
  source 1..2690: mol_type = other RNA
gctgggattacaggcatgagccactgcgcccagcccctgttcatttttttatgtgtggcccaagacaattcttcttccaatgtagcccagggaagccaaaagattagacgcccctgcttagcatatcctgggtctccctcactcctcgcaatccatcgctgtcccccagggcctccagctgcagcacctctctgtcctgcagccatttacctcatgctcctccctgactgctggactgaggctctgtgaggtcagggcctggcccagacatggctcaatggatgctcaatagaaaggctggatgttggaggtgtgaggacagccagctccactccatcccacagctgtctcctgcagcaacctttctgcaccccctggctcctcctcctgtcattcattcattcaactcatttgttcaactcctgtcatccactcatccaacaaacatagaggacttagcctgtgtcaggctctgactttcagttgggatggaagacagcgtccttacatggacacttggatgactaaggaaggaacttagtaggtgccaaagtgaccctaaggtaggtgcaacctttctgcaccccctggctcctcctcctgtcattcattcattcaactcatttgttcaactcctgtcattcactcatccaacaaacatagaggacttagcctgtgtcaggctctgactttcagttgggatggaagacagcgtccttacatggacacttggatgactaaggaaggaacttagtaggtgccaaagtgaccctaaggtaggtggcctgaggccagcaggtatcctgtgaaaacaatggcagagactcaggctcccatactgggagtcatattattggtgtgcagtacaaaatcactgacaaaacacacctgtgcccatgagccaagcatgcaaagggccaaaggtgtctgctggaatttcttcaaagaggcagctctgtgcgagcactgagcatgcacacttgtggacccctgtcctgggcgaggaccatgcctgagttcttctgctaggagatccaccctctctcccaaatcactcaccagaggttctcccctctgcccaggctcataaagatttgagagctcagccaggtgcggtggctcacgcctgctaatcccagcactttgggaggccgaggcaggcggatcacgaggtcaggagttcgagaccagcctggccaacattgtgaaaccctgtctctactaaaaatacaaaaattagccaggcgtagtggtgcgcacctgtagtcccagctactcaggaggctgaggcaaaagaatcgcttgaaccctggaggcagaggttgcagtgagctgagatcgtgccacggcactccagcctgggcaagagagcgacactccgtctcaaaaaaaaaaacaaaaaaaaaaacacaaagatttgcgagctcagagacaaaggaaatgccatgtgttttccccttcttctgagccccgtggggccagagcacgccttcctctgccttggcaatgacagacaagctggggtccttccccattgccagctctgcagcactgccctcctgggaaccacattcagtcattctgtggagttttcatgatgggtttcatcatcagattcatttcctccatgggagtagactcttcagcaagtcacattacctctccgggcctcagtttcccctcttgtgaaacaacagggtagaacttaagggcccttcctgttttctctgacagtctgaatctgtcttgtgcacgtacatagccctgcaatagtgtcaaagatctttaattgttggatggaaaagaaaggaacctgtgggttttgaggggggacaggtaccgccaaatgcagatgatgattctgagagcacctttgacgggccagatctcgtactctgagtttatctgcgccacttgttgtctggcaagtccagtgatgctgtggtctccagctgattctatctgagctgctcctggggtggcagctctcagaagtgtgggagaggatgcaggcgatggggagggaccgggaccgcatgctccctccaggacatagcgcacaacggtggtctggggtaggatgaagtataagtgctctgcttcaggccagccttgggtgtgagctgtctctgcttgagctgctcatagagtccatagtttgtagggggagcaagaaggggaaagtcagacttctctggcagccacagcaacttctgtccattccaagtgcggagtggaggcagccccgggttgtaaccatgccggttgtaatggtcgtcataggtgctgatcaggtagcgatgtgggggctcctggtggtgggtgatcaggtgtttgtaaggtagcccctttctcctctcttccatccaatttccagtgagcactttcgttgaatacttggtctcaatctgccagctcggagtagagagtggctgtggatttactgcagtcaaaaacatgttaaggatttgccccaggtttctttgacttgatgcagtttaaggcttcaggcggggagaggaaggtgttatgaagttgctgagtttggggtgcctattttgtcttcccagctggcctcctgaatggctagtagatgactccttgctaacctcagagaataaaacggccccaagagttcactgtcagcctttagggagagttgatctatcttggattctctactgttgact

SEQ ID NO: 15291 - RNA, 1448 nt, Homo sapiens
  source 1..1448: mol_type = other RNA
gctgggattacaggcatgagccactgcgcccagccgagagttttaaagaaggtgaaagctcttcccttttcctaacctagcttggccttgattctattaataccaagcctgtgtgaattggagtggaaagcagaagtgctgaagggagccattgccagagggaagaacacaaacttcaaggccagatgctcagcggagctctcagaacagccaagccaggaggacagtcaggaggaccataggccaggccaccaggaaccctgcagtgctaggggttccattcatgacaccgggagactgtgcacctctccgagtgatgggccccaaatctagaacccgggctaggtcgatggccggtacttcactgcggacttgacttcttgagcaagaaggctggcactgttcattaagagaatcacagagatgaatctcacaatgcaggaaaactaggtcataatgtccagcaaacatgaacatctgaactgagaaccggctttccgaggactgcccattctcctccacgtggatggtggaatcacgttgatttgagcagctgtttctgatgatgaaatacttcacaaggtcagccttgtcttcagtgggggtggcatagcagttcctcaacaccaggttaaaccgggaggtgtccccttgttccaagatggcacccacatacagcacggactcaacagacagttcaactgcatccccttcgtaaggattcgtgtagttctggtcttggaagagggccatcctgacaatgaactctccattcccgtccacactgacgttcagggaacttacaatgggctgcaaggcagcttggaggctgactttcatgtccagtgggtaggcacattggaagttgatgttgaggatggtgtctctgatgatgaaatcattgaccaaggagagggtgtttttgtagatggcatgggtttgatttctctccagaatgttcctgcaggcactagcctggacggggctggtcacagatacccagttcctctcctctgtctgcaagatgctgctgcagtttgggtctcgcaggtaggcaatgacctcctcccccaaacccaggcctcccagcaaacatttgtccaccttcaccttgatctccctgggcccacagtctagctgaggctgcaaactgtggacatcagaactattgaggtcctgtctgcagaaacagccccaggtgctgttgagggcaaggcactcctcctcggggcggcaggccttctcacacttgtcctccacagtggatgggtctcgctgcactgcagatgcctgggtcagaatgcaggagaccaaggccagccacaggaggccagagcccaccatcctttccataaggtgaggcatgcaggtcactttgctgtatgcagacttcccatgcagctccgatgagaacacaaagcgttcctcctctggccagccatgggaat

SEQ ID NO: 15292 - RNA, 1457 nt, Homo sapiens
  source 1..1457: mol_type = other RNA
gctgggattacaggcatgagccactgcgcccagccgagagttttaaagaaggtgaaagctcttcccttttcctaacctagcttggccttgattctattaataccaagcctgtgtgaattggagtggaaagcagaagtgctgaagggagccattgccagagggaagaacacaaacttcaaggccagatgctcagcggagctctcagaacagccaagccaggaggacagtcaggaggaccataggccaggccaccaggaaccctgcagtgctaggggttccattcatgacaccgggagactgtgcacctctccgagtgatgggccccaaatctagaacccgggctaggtcgatggccggtacttcactgcggacttgacttcttgagcaagaaggctggcactgttcattaagagaatcacagagatgaatctcacaatgcaggaaaactaggtcataatgtccagcaaacatgaacatctgaactgagaaccggctttccgaggactgcccattctcctccacgtggatggtggaatcacgttgatttgagcagctgtttctgatgatgaaatacttcacaaggtcagccttgtcttcagtgggggtggcatagcagttcctcaacaccaggttaaaccgggaggtgtccccttgttccaagatggcacccacatacagcacggactcaacagacagttcaactgcatccccttcgtaaggattcgtgtagttctggtcttggaagagggccatcctgacaatgaactctccattcccgtccacactgacgttcagggaacttacaatgggctgcaaggcagcttggaggctgactttcatgtccagtgggtaggcacattggaagttgatgttgaggatggtgtctctgatgatgaaatcattgaccaaggagagggtgtttttgtagatggcatgggtttgatttctctccagaatgttcctgcaggcactagcctggacggggctggtcacagatacccagttcctctcctctgtctgcaagatgctgctgcagtttgggtctcgcaggtaggcaatgacctcctcccccaaacccaggcctcccagcaaacatttgtccaccttcaccttgatctccctgggcccacagtctagctgaggctgcaaactgtggacatcagaactattgaggtcctgtctgcagaaacagccccaggtgctgttgagggcaaggcactcctcctcggggcggcaggccttctcacacttgtcctccacagtggatgggtctcgtggaactcgctgcactgcagatgcctgggtcagaatgcaggagaccaaggccagccacaggaggccagagcccaccatcctttccataaggtgaggcatgcaggtcactttgctgtatgcagacttcccatgcagctccgatgagaacacaaagcgttcctcctctggccagccatgggaat

SEQ ID NO: 15293 - RNA, 1898 nt, Homo sapiens
  source 1..1898: mol_type = other RNA
gctgggattacaggcatgagccactgcgcccagccgagagttttaaagaaggtgaaagctcttcccttttcctaacctagcttggccttgattctattaataccaagcctgtgtgaattggagtggaaagcagaagtgctgaagggagccattgccagagggaagaacacaaacttcaaggccagatgctcagcggagctctcagaacagccaagccaggaggacagtcaggaggaccataggccaggccaccaggaaccctgcagtgctaggggttccattcatgacaccgggagactgtgcacctctccgagtgatgggccccaaatctagaacccgggctaggtcgatggccggtacttcactgcggacttgacttcttgagcaagaaggctggcactgttcattaagagaatcacagagatgaatctcacaatgcaggaaaactaggtcataatgtccagcaaacatgaacatctgaactgagaaccggctttccgaggactgcccattctcctccacgtggatggtggaatcacgttgatttgagcagctgtttctgatgatgaaatacttcacaaggtcagccttgtcttcagtgggggtggcatagcagttcctcaacaccaggttaaaccgggaggtgtccccttgttccaagatggcacccacatacagcacggactcaacagacagttcaactgcatccccttcgtaaggattcgtgtagttctggtcttggaagagggccatcctgacaatgaactctccattcccgtccacactgacgttcagggaacttacaatgggctgcaaggcagcttggaggctgactttcatgtccagtgggtaggcacattggaagttgatgttgaggatggtgtctctgatgatgaaatcattgaccaaggagagggtgtttttgtagatggcatgggtttgatttctctccagaatgttcctgcaggcactagcctggacggggctggtcacagatacccagttcctctcctctgtctgcaagatgctgctgcagtttgggtctcgcaggtaggcaatgacctcctcccccaaacccaggcctcccagcaaacatttgtccaccttcaccttgatctccctgggcccacagtctagctgaggctgcaaactgtggacatcagaactattgaggtcctgtctgcagaaacagccccaggtgctgttgagggcaaggcactcctcctcggggcggcaggccttctcacacttgtcctccacagtggatgggtctcgtggaactgtgcagtatctcagattacaccagggagtgccttccaaccggtacacatggtacccgcctgggcaggccttcaccagcacctctgttttccagaaacagcagttgccactccaatgggcacaggcagtgtggttggtgatgccatccccaagggcagggtgggtcccattcagccacatgggagcgtctgtctggcatcggtgcacctggacacaggtctccgacatccttactcctccttcccctacaaagcggtaccagccgctcatgtttttatcgcacccctgggaccctgctgagttctctgtgcttcggaagggttcatccaggagggtgtaattctgacaggggtcaaaacagacatgagcctctggggtgccaggagctccgcagtccaggtccagcccatacgaactggcttcaatggggtttccataacctcgctgcactgcagatgcctgggtcagaatgcaggagaccaaggccagccacaggaggccagagcccaccatcctttccataaggtgaggcatgcaggtcactttgctgtatgcagacttcccatgcagctccgatgagaacacaaagcgttcctcctctggccagccatgggaat

SEQ ID NO: 15294 - RNA, 1889 nt, Homo sapiens
  source 1..1889: mol_type = other RNA
gctgggattacaggcatgagccactgcgcccagccgagagttttaaagaaggtgaaagctcttcccttttcctaacctagcttggccttgattctattaataccaagcctgtgtgaattggagtggaaagcagaagtgctgaagggagccattgccagagggaagaacacaaacttcaaggccagatgctcagcggagctctcagaacagccaagccaggaggacagtcaggaggaccataggccaggccaccaggaaccctgcagtgctaggggttccattcatgacaccgggagactgtgcacctctccgagtgatgggccccaaatctagaacccgggctaggtcgatggccggtacttcactgcggacttgacttcttgagcaagaaggctggcactgttcattaagagaatcacagagatgaatctcacaatgcaggaaaactaggtcataatgtccagcaaacatgaacatctgaactgagaaccggctttccgaggactgcccattctcctccacgtggatggtggaatcacgttgatttgagcagctgtttctgatgatgaaatacttcacaaggtcagccttgtcttcagtgggggtggcatagcagttcctcaacaccaggttaaaccgggaggtgtccccttgttccaagatggcacccacatacagcacggactcaacagacagttcaactgcatccccttcgtaaggattcgtgtagttctggtcttggaagagggccatcctgacaatgaactctccattcccgtccacactgacgttcagggaacttacaatgggctgcaaggcagcttggaggctgactttcatgtccagtgggtaggcacattggaagttgatgttgaggatggtgtctctgatgatgaaatcattgaccaaggagagggtgtttttgtagatggcatgggtttgatttctctccagaatgttcctgcaggcactagcctggacggggctggtcacagatacccagttcctctcctctgtctgcaagatgctgctgcagtttgggtctcgcaggtaggcaatgacctcctcccccaaacccaggcctcccagcaaacatttgtccaccttcaccttgatctccctgggcccacagtctagctgaggctgcaaactgtggacatcagaactattgaggtcctgtctgcagaaacagccccaggtgctgttgagggcaaggcactcctcctcggggcggcaggccttctcacacttgtcctccacagtggatgggtctgtgcagtatctcagattacaccagggagtgccttccaaccggtacacatggtacccgcctgggcaggccttcaccagcacctctgttttccagaaacagcagttgccactccaatgggcacaggcagtgtggttggtgatgccatccccaagggcagggtgggtcccattcagccacatgggagcgtctgtctggcatcggtgcacctggacacaggtctccgacatccttactcctccttcccctacaaagcggtaccagccgctcatgtttttatcgcacccctgggaccctgctgagttctctgtgcttcggaagggttcatccaggagggtgtaattctgacaggggtcaaaacagacatgagcctctggggtgccaggagctccgcagtccaggtccagcccatacgaactggcttcaatggggtttccataacctcgctgcactgcagatgcctgggtcagaatgcaggagaccaaggccagccacaggaggccagagcccaccatcctttccataaggtgaggcatgcaggtcactttgctgtatgcagacttcccatgcagctccgatgagaacacaaagcgttcctcctctggccagccatgggaat

SEQ ID NO: 15295 - RNA, 7911 nt, Homo sapiens
  source 1..7911: mol_type = other RNA
gctgggattacaggcatgagccactgcgcccagcctacactgctttcttaagtgggtccccagtcatgttctcctcactgggtaagacctttcaacaggggtttccagctacctcctacagttgctttggggctggaaaccggtctatacctcccttagatggagctcttagaaaaaagggcatgctgccattgttgctgttttacagtattcactggtgataatgttgtcaggtactggaaaatctgaggtgactagaaactgcagtggacacccagcatactgcagcagcccttcagaaaagtggccagactgttacgtgagtgcctgttctcatatattctcactgggcaagttctccaggcctgggccactagccaatcattgccagagctattgagccagtagcaacttcgcaactccctagacagagcctccaagagcaactgaaaatatttttgccattgcctctgcagtagaactgtccttgctaccctcagactaatgaaaaatccaacaccctaagtgccttattcacacctcaaacgagctgtagtttacccaaggagagagggccagtccatcctccatgggtcccacaaactacccactgctcattaccagtgaacccctaatttggccaaaagcacagatcctccatcctggtcggactgcactgagtgattgctggcctacacgtctctgagatgcagcaaccagaagacaggcaaagaggtggggcagcaacccagctcatgtggtacccagagggtttagtgcaagagcacctgtagtagagtgtggccattgacggccatttccataggctcaactttctcccataagagactttagccctaggggaactgttggacctaatttctgcaggatggtcttgcaaatcagaagaagctgatccaactgagcactccttggtctgctggcctctcccagggatccagtctggccacaactgcttacagggcagtctcaggtaccctaggagcccataccatagcatctgcactggtgggccatgcctgacccatgaagagctccggcaaggcagcccctgtgactgcaccagctcacatgtttcttccctatactccagcttcccccaagaccatggcaactccccatattactttgctggcacatgtctgcaaaggtgagtttggctttgcttgccccaccagaaaatggaaatgtagtatgcccctgccactcccagcaattgctattgtagatgaagctttggcgggtagagagccagaaagccccaccctggcctttgtggtaaaactgtgcggagaacagggtatcctcccacactctgaacaatcattccttcttggggggcacagagaaggcatcaaaacctttactggccagtatcctgccccaagccaacaccacctttagtgaaatagcacacagtctccagcaggtaacccccactcccctcccagctgctttgctcctgccactgaagtgaatacccaaagacaggcagaaaccccatatccactagcactctgcagcagctgtggcaccttagtcccacagagtggcagactccaaatcacaaggagccacagaacacagttggggctcaatacaactcccccagagttagagtatgcagactctaagttgtgagctgagcatttagagtatgcagcctctgagttgtgagctgagcattgccccctccaccaccacaaaaaaaaaaacaaaaacaaaaaacaaaaaacaaaaaactcccaggaacaaagcctgttggctgaatccaccttttaccacaatcaaatactcaagaccatcaaataggatccaaaaaaccaaaccccattcaaagttcagcaactttaaagatacgcccacaaagatgagacaaaatcagtgcaaaaatgttgaaaacacaaaaagccagagtgacttctttcatccaaatgaccaaattacattaccagcaaggcctaagatgacagaagcagaattcagaatatgggtagaagcaaacttcattgatctacaaaggtaagttgcaacccaatgcaaagaagaaaaaaataattgcaggaagtgatggaaaaaacagccagtctagagaaaaatatggccaacatgatagaactgaaaaacacaatacaaaacctttataatgtaatcacaagtgttaatagaagaataggccaagcagagggaagaatctcagagcttcaagactggctttctgaaataagacagacaagaatagtgaaaaaagtataaagaggaatgaacaaaacctccaagaaataacagattatgtaaataaaccaaatctataattaaagagagtgcttgaaagtgatggagagaatgaaaacaacttgaaatacatatttcgggataccatccatgagaatttccccaaactagagaggccaacattcaaaggcaagaaatgtggagaaccccaataatataccccacgagaaggtcatccccaagatacataatcatgagattctccaaggtcaaaatgagagaaaaaaatatgttaaaggcagctagagagaaagaccaggtcacctctaaaaagaagctcagacaacaatgaaccttgcagctgagatccctcaagtcaaaagagattaatggccaatattcaactttctttaaaaaagaattctaatccagaagttcacatccggccaaagtaagcttcagaagcaaaaaataaatatgatcgtattcagataagcaaatgctgaggaaatctgttaccacaagacctgccttaaaagatcttctgaagaaagccctaaataagaaaaagactataaacagtcactacaaaaacacactaaagtacacaaaccactgacatgataaagccaccacataaacaaatgtgcaaaatagccagctaagatgatcatgacagaatcaaatccacacatatgaatacaaaccttaaatgtacatgggttaaatgcccaaattaaaaaacagagtggcaaataaagaaccaagatctaatggtatgctgtaattgagatacccatttcaaataagctcaaaataaagggaaaagtctaccaagcaaatagaaaacagtaaaaaagcaaggattacaatcctagtttctgacaaaacagactttaaatcaacagatttttttaaaaagacaaaaaatggcattacataatagtaaagggctatatatgcatccaacacaaaagcacccagttatgaagcaagttcttagagaccctctaagatgttattaaatgttcttcaagtcattacctttatactacatttgttcagtagtaagtctctgatgttgaacacaatatgacgaattgttaaaggcttttccacatttttaacacttgtggagcttctctctactatgaattgtcttatgtctaatgacgtgtgagaacgagctcaatactttgccacattcttcacatttgtagggtttctcaccagggtgaattctcttatgattagtaaagtctgagagccacataaaggttttgccacattcttcgcatttgtaaggtccctcttccatatgaattctcttgtggttaataaggattgaggagtaggtaaaggccttgccacattcttcatggatgtagggtgtctctccagtatgaattctcttatgttttctaagggccgagatccacataaaaccttttccacattcattacatttgtagggtttctctccaatatgaattatcttatgtttagcaaggtctcagaaccacctatagcctttgttacattcttcagatttgtagggattctctccagggtgaattctcttttgattagtcaggtctgagaaacacaggttttgccgcattcttcacatttgtaaggtctctcttccatatgaattctcttgtggcttgtaagggttgaggagcggataaaggctttgccacattcttcacaaatgtagggtttctctccagtatgaattctcttgtgtttactaagggccaagatccacgtaaaagcttttccacattcattacatttgtaaggtttatctccagtatgaattaccttatgtttagtaaggtctgagaaccacctaaaggctttgccacattctttgcacttgtaggtctgtctccagtatgacttctcttgtgtttaataaggcttgaggagcaggtaaaggttttgccacattcttcacatttgtagggcttctctccagtgtgaattctcttatgattagtcaggtctgggaaccacttaaaggttttgccacattcttcacatttgtaaggtctcacttccatatgaattctcttgtgtttaataaggtttgaggagcaggtaaagcttttgccacattcttcacatttgtagggtttctctccagtgtgaattctcttatgattagtcaggtctgagaaccacttaaaggttttgccacattcttcacatttgtaaggtctcaattccatatgaattctcttgtggctaataagggttgaggagtaggtaaaggctttgccacattcttcacaaatgtagggtttctctccagtatgaattctgttatgttgactaagggccgagatccacataaaagcttttccacattcattacatttgtagggtttctctccagtatgaattctcttatgtttagtaaggtctgagcaacacctaaaggctttgtgacattctttacatttgtagggtttctctccagtatgaattctcttatgtttagtaaggtctgagcaacacctaaaggctttgtgacattcttcgcatttgtagggtctgtctccagtatgatttctcttgtgtttagtaagggctgaggaacaggtaaatgttttgccacattcttcacatttgtagggtttctttccagtatgaactctattatgttcagtaaggtttgagaactttttacaggctttgccacattcttcacatttgtaacttctatctgcagtatgaattctcttctgtatggtaaaatctgacaacctacagtctttgccacattcttcacatttgtagcatttctctctgctaaaaattttcttatgttcagtgaagattgagcacaacccaaaagctttgccacatttattatattgacaggttttgctacgggtagctgacaaacattgatgaatgccattataactgcttttctgccccttgcaattacccacacgttggtagtctttctttaaacgtaaagtattaaggtcacagcttccagattttctcaggatcactttttgaaatgaatcgtttatgtcgtgctccagcaatatctctgcagtaaaatgcaaagagccagccaaggagaacaggtttccgtagttctctaacatcacatccctatacaaacgctgctgagcagagtccaggcattcccactcttctggggagaattctacagccacatccctgaatgttagcactcgcatttcccagcctccggatgttccgccttcttccctatggatctcccagtacctgcaggtcacaggataacaggggctatggtggagtcaccgaggagctaatggagcggaagagatggaatagtacagacgggtactggactcagagcctagaagctaggagacgaaggccttgccatattgaagagcccgcctcttcctctctagctgcgcacctgattgggcagttttcacgctagcaccactgattggctggggttctccgccccacacatttagaccctgatcgacaggagatgtaatgagacactgggctgaatgaggaaagagtgacaggtttttgcctgcagcatgttcaggcagcgatttctccttgtgttgggggcctggccctgcctgagggacatttgtatttaacgttgtatataagattatatcactttctgattatatttacgtgtgtgtatatcaatttctgaattatagttatgtgtatgctgcaggccctgtctcagcatcctgtctttccctttagttgcaggagatcaaagtcctccaggagatgcagctgcaccagctggctgcagacaattatcaccttcagtctgtgaagcaattttgggtctgcttccaattaatggagtgtctcagtgagactgagaggtgagggcctagcagattggttagtgccactcacccagacctcccaaaacaccctgtttctttcccaccaaagctgagcctgcctgaggacctaaacaagcatggagaacgaagatgggaccctagtcagggatagtgctgggctgtggggtaaagtcagctgggtcagtgcctccaggtgtgggaaggagccggcctcttctctagggccctgggcaagtcactgccctctttgggcctctgttttcttatccaaaaaatgtagggatgatgagactgagaggggctaatgatgagcttcaaaggagaaaagaactttgagagtgcttgtgcctggctcttcctgagatgatgagaacaatggtgacagctacatataactgagtcctcacaaggcccagtgaggtaggtggttcccatcacactttcaagttgagaaaacagtctcagggaggcctggctgcatgcccaaggttccacatacagggagtgttggagcagggagtcaatctagaatcagaacttactggagatgacaggagcattggaccagcttactcacaccagttatccaggataccaggtcagtgtaactgggcataactgggtgaagggagcatagtatcactgaccttttctttgactctggcagatgaagacatccacgttggccaccctggagacgaaaccacagagaggccagatgaggctaaagcagcaaaaaggcagtgtccctgtgatggggaggagctccagggagtcagagggaagagctcctccctcacagccggaggcctccacatcaaaagagcaaggggcctttctcccgtagcccttccctcctgtggcaacagtccctgaaatgcctctataagacaaatctgagtaaaagcctggaagagctggatttgggaaatagtgggggcagggaccacataacattgtgacttgtaaaaatctcaccacagagttaacatgggaacatgggggttcatgtttttggaggccagctaggaggaggggagagagttggggagaggcagctgagtgtctttggctttttcaagtggaagatgtagataggagggtccaggagacaggggattatgagacttcaggggacaggccttgaatggacacccaaaattggatactcatccccatcaccacccgatggcacagggtgttgcctccatcctgggcacattttccagttatctggtgatgggagaccctgccagaaaggattatatggatgggagtgagcctgggatgggcagggctggaaccaggatcctgaggcttgggaaaagagaatccaggactacacccttagatctcagcacttggcaaacctcctctcatgagagcctcacggctgcctctgtgagctgaggcatcaggcccctcttccctatgaatgttgaagattccacatcagccgtcagtccctgttcccagagtggtgaagctgcagagctgcctgcttgcaaagctcagtgaggtttggcctgagctggactcagactctccctcaggtggttccaatggaaggagagtaaacttagacctctctaagggcaggcagctcatataagcctgagcacttttttaatgggagcctccagtttttctgtcatcagagagagttggggcgggaggtccctgagcctcagctcccattgttctgttctttgaaccccagaacctgctgcagacccaactcctgctttgtgcacatgccctgaccctggtggccctggcagta

SEQ ID NO: 15296 - RNA, 5767 nt, Homo sapiens
  source 1..5767: mol_type = other RNA
gctgggattacaggcatgagccactgcgcccagcctacactgctttcttaagtgggtccccagtcatgttctcctcactgggtaagacctttcaacaggggtttccagctacctcctacagttgctttggggctggaaaccggtctatacctcccttagatggagctcttagaaaaaagggcatgctgccattgttgctgttttacagtattcactggtgataatgttgtcaggtactggaaaatctgaggtgactagaaactgcagtggacacccagcatactgcagcagcccttcagaaaagtggccagactgttacgtgagtgcctgttctcatatattctcactgggcaagttctccaggcctgggccactagccaatcattgccagagctattgagccagtagcaacttcgcaactccctagacagagcctccaagagcaactgaaaatatttttgccattgcctctgcagtagaactgtccttgctaccctcagactaatgaaaaatccaacaccctaagtgccttattcacacctcaaacgagctgtagtttacccaaggagagagggccagtccatcctccatgggtcccacaaactacccactgctcattaccagtgaacccctaatttggccaaaagcacagatcctccatcctggtcggactgcactgagtgattgctggcctacacgtctctgagatgcagcaaccagaagacaggcaaagaggtggggcagcaacccagctcatgtggtacccagagggtttagtgcaagagcacctgtagtagagtgtggccattgacggccatttccataggctcaactttctcccataagagactttagccctaggggaactgttggacctaatttctgcaggatggtcttgcaaatcagaagaagctgatccaactgagcactccttggtctgctggcctctcccagggatccagtctggccacaactgcttacagggcagtctcaggtaccctaggagcccataccatagcatctgcactggtgggccatgcctgacccatgaagagctccggcaaggcagcccctgtgactgcaccagctcacatgtttcttccctatactccagcttcccccaagaccatggcaactccccatattactttgctggcacatgtctgcaaaggtgagtttggctttgcttgccccaccagaaaatggaaatgtagtatgcccctgccactcccagcaattgctattgtagatgaagctttggcgggtagagagccagaaagccccaccctggcctttgtggtaaaactgtgcggagaacagggtatcctcccacactctgaacaatcattccttcttggggggcacagagaaggcatcaaaacctttactggccagtatcctgccccaagccaacaccacctttagtgaaatagcacacagtctccagcaggtaacccccactcccctcccagctgctttgctcctgccactgaagtgaatacccaaagacaggcagaaaccccatatccactagcactctgcagcagctgtggcaccttagtcccacagagtggcagactccaaatcacaaggagccacagaacacagttggggctcaatacaactcccccagagttagagtatgcagactctaagttgtgagctgagcatttagagtatgcagcctctgagttgtgagctgagcattgccccctccaccaccacaaaaaaaaaaacaaaaacaaaaaacaaaaaacaaaaaactcccaggaacaaagcctgttggctgaatccaccttttaccacaatcaaatactcaagaccatcaaataggatccaaaaaaccaaaccccattcaaagttcagcaactttaaagatacgcccacaaagatgagacaaaatcagtgcaaaaatgttgaaaacacaaaaagccagagtgacttctttcatccaaatgaccaaattacattaccagcaaggcctaagatgacagaagcagaattcagaatatgggtagaagcaaacttcattgatctacaaaggtaagttgcaacccaatgcaaagaagaaaaaaataattgcaggaagtgatggaaaaaacagccagtctagagaaaaatatggccaacatgatagaactgaaaaacacaatacaaaacctttataatgtaatcacaagtgttaatagaagaataggccaagcagagggaagaatctcagagcttcaagactggctttctgaaataagacagacaagaatagtgaaaaaagtataaagaggaatgaacaaaacctccaagaaataacagattatgtaaataaaccaaatctataattaaagagagtgcttgaaagtgatggagagaatgaaaacaacttgaaatacatatttcgggataccatccatgagaatttccccaaactagagaggccaacattcaaaggcaagaaatgtggagaaccccaataatataccccacgagaaggtcatccccaagatacataatcatgagattctccaaggtcaaaatgagagaaaaaaatatgttaaaggcagctagagagaaagaccaggtcacctctaaaaagaagctcagacaacaatgaaccttgcagctgagatccctcaagtcaaaagagattaatggccaatattcaactttctttaaaaaagaattctaatccagaagttcacatccggccaaagtaagcttcagaagcaaaaaataaatatgatcgtattcagataagcaaatgctgaggaaatctgttaccacaagacctgccttaaaagatcttctgaagaaagccctaaataagaaaaagactataaacagtcactacaaaaacacactaaagtacacaaaccactgacatgataaagccaccacataaacaaatgtgcaaaatagccagctaagatgatcatgacagaatcaaatccacacatatgaatacaaaccttaaatgtacatgggttaaatgcccaaattaaaaaacagagtggcaaataaagaaccaagatctaatggtatgctgtaattgagatacccatttcaaataagctcaaaataaagggaaaagtctaccaagcaaatagaaaacagtaaaaaagcaaggattacaatcctagtttctgacaaaacagactttaaatcaacagatttttttaaaaagacaaaaaatggcattacataatagtaaagggctatatatgcatccaacacaaaagcacccagttatgaagcaagttcttagagaccctctaagatgttattaaatgttcttcaagtcattacctttatactacatttgttcagtagtaagtctctgatgttgaacacaatatgacgaattgttaaaggcttttccacatttttaacacttgtggagcttctctctactatgaattgtcttatgtctaatgacgtgtgagaacgagctcaatactttgccacattcttcacatttgtagggtttctcaccagggtgaattctcttatgattagtaaagtctgagagccacataaaggttttgccacattcttcgcatttgtaaggtccctcttccatatgaattctcttgtggttaataaggattgaggagtaggtaaaggccttgccacattcttcatggatgtagggtgtctctccagtatgaattctcttatgttttctaagggccgagatccacataaaaccttttccacattcattacatttgtagggtttctctccaatatgaattatcttatgtttagcaaggtctcagaaccacctatagcctttgttacattcttcagatttgtagggattctctccagggtgaattctcttttgattagtcaggtctgagaaacacaggttttgccgcattcttcacatttgtaaggtctctcttccatatgaattctcttgtggcttgtaagggttgaggagcggataaaggctttgccacattcttcacaaatgtagggtttctctccagtatgaattctcttgtgtttactaagggccaagatccacgtaaaagcttttccacattcattacatttgtaaggtttatctccagtatgaattaccttatgtttagtaaggtctgagaaccacctaaaggctttgccacattctttgcacttgtaggtctgtctccagtatgacttctcttgtgtttaataaggcttgaggagcaggtaaaggttttgccacattcttcacatttgtagggcttctctccagtgtgaattctcttatgattagtcaggtctgggaaccacttaaaggttttgccacattcttcacatttgtaaggtctcacttccatatgaattctcttgtgtttaataaggtttgaggagcaggtaaagcttttgccacattcttcacatttgtagggtttctctccagtgtgaattctcttatgattagtcaggtctgagaaccacttaaaggttttgccacattcttcacatttgtaaggtctcaattccatatgaattctcttgtggctaataagggttgaggagtaggtaaaggctttgccacattcttcacaaatgtagggtttctctccagtatgaattctgttatgttgactaagggccgagatccacataaaagcttttccacattcattacatttgtagggtttctctccagtatgaattctcttatgtttagtaaggtctgagcaacacctaaaggctttgtgacattctttacatttgtagggtttctctccagtatgaattctcttatgtttagtaaggtctgagcaacacctaaaggctttgtgacattcttcgcatttgtagggtctgtctccagtatgatttctcttgtgtttagtaagggctgaggaacaggtaaatgttttgccacattcttcacatttgtagggtttctttccagtatgaactctattatgttcagtaaggtttgagaactttttacaggctttgccacattcttcacatttgtaacttctatctgcagtatgaattctcttctgtatggtaaaatctgacaacctacagtctttgccacattcttcacatttgtagcatttctctctgctaaaaattttcttatgttcagtgaagattgagcacaacccaaaagctttgccacatttattatattgacaggttttgctacgggtagctgacaaacattgatgaatgccattataactgcttttctgccccttgcaattacccacacgttggtagtctttctttaaacgtaaagtattaaggtcacagcttccagattttctcaggatcactttttgaaatgaatcgtttatgtcgtgctccagcaatatctctgcagtaaaatgcaaagagccagctgggtgtttggctactgtcttctgtctcctcgcattccaaggctcttttctttgctccagataggtaatcaagtctggcttaaagatagcaagacccaaggagaacaggtttccgtagttctctaacatcacatccctatacaaacgctgctgagcagagtccaggcattcccactcttctggggagaattctacagccacatccctgaatgttagcactcgcatttcccagcctccggatgttccgccttcttccctatggatctcccagtacctgcaggtcacaggataacaggggctatggtggagtcaccgaggagctaatggagcggaagagatggaatagtacagacgggtactggactcagagcctagaagctaggagacgaaggccttgccatattgaagagccc

SEQ ID NO: 15297 - RNA, 2434 nt, Homo sapiens
  source 1..2434: mol_type = other RNA
gctgggattacaggcatgagccactgcgcccagcctgctgggaacattttaaggttcaattaatgcatgctgcttaggtaactatgattaaaatgtatacgttagcatagaactgataataattgagctttagttacagcatttcctttctcctaacatctcccttacccagaaacaacttaaaacacttcaaattttttgagttagagatcacaaacatcaaggtatttgactcttattttccatcacttgctacttgagggggtcacactaaccaattctggttacatactttcctgctatggactctagaagaaaaactgcaaagaaacagaaaactaaccttcttaaacatatataaggaatcaagggtttccttaaactattacctgagagtcctatttttgccttctgtatagtaagcatgtcattctactcactattctgccggaatacatcttcacatttcaaactggattactttccaaatactggattacgttcatgcagtaaaaacaagaatagtgcatctattgaatatttttgcatttgcttattgcaatactagttaaaacaccagtttataatttttttatacattcagttgttcaacaaatgattcttttaatctgcctgaagtttcaagtcaacacgtcactggagaaaatgtatgaaactgtagcactaatttctgaaacgaaggattgaagttcctctttccaacttctttcagaccatcactactccacatgttcctgctcttgtcctggaattagccaccgaatactctcagttcgaatggtagcatacataataaaactaattaaaaagaataaggaaaatacaagcaaccagtccacactttttatcaaagtgctgggaagagggcctatttggtcggcttgagttaccaccacattcttcttggcttctatacctgtctgattaaaaatgaagattttcagtgtttccagtgttcgatctgtatgattaaatctggccattggtttagctccttgaaataataaaatattaggaacagctacggtgccaaacctggtagaaaggctgctgtgctgagatgcatccagtgccaaaaagtgaagagctggaaatgcccggggcagagagttaaagtgaggggccaaactggcagaaaagcggcaccacggggtgtaaaacaggactagagtacagtcactaccgtttgggttcagaaaatccataaggtcctgtgacatatttaaaattttcagagtgaaattttctaatcctgtaatgtttctctcctcacagttcacctttggggatttcagactttcagtgttattggagtcctctgtcggggctgcgtcagattccgccacttctggctctgtgtaatactcctcttctctgtcagggaagtgtgctccagcgccatccagagagaaaaggctctctcggacgttgcaccttgagtcctccgctcctccagcaccacaggtgacgccgctaggctctgaactcactttgtcctcagcttccccaggaatcacagacagcatcaccatgtgatcgccttgggtgtccagccccagcaccgcattggcctcttctgctgccctgtcctggcccatcgggtcatgcaggagctcctcctcacccaggtacacagcccccacctggagagggtgagcaggctgctcctctgaccataagcgaccactttcctctgcaacaccagccgaggagccgcatgacgcggggcggtcgtcgaccggcagccgggaccattgcccaggccgagaggcaatcggcgcacggctacgcgagtcgtgctgccagccggaggaaggctgggggaggagagcctgggagcgcgggcgcggccccgcgccgccatcttaacacctggcagctgtggcgggcgccatcttggagtcgggcggacggcctctagccgctggccgtcggcgctggactggagacctctttaggagctaagcgccagacgttgcaggtcgttttgaactctgctgaccccagagtgcagagcatggctctggcagaggcccatggcctcctttcttccctcggaagtcagagcttggctacttgaagcactgcgcccgcctaaggagggttttccacgcttcattcccagagccagaaaggcccaggagccttcctgttctagtgtcccatcgaggtgcagaaactttggaggctgcaaatcttctaatcgcttgcctaacctgtgctcccctacctagggttgccacatagaatacctgatacccagttatatttgaatttcacataatgaatattttttactataacccttatagtataagggatataccttaaaactgagcatcctgtaacttcgtgacatctggcaaccctaaccctacctatccactcagggcaggagaggttggttttaact

SEQ ID NO: 15298 - RNA, 1880 nt, Homo sapiens
  source 1..1880: mol_type = other RNA
gctgggattacaggcatgagccactgcgcccagcctgctgggaacattttaaggttcaattaatgcatgctgcttaggtaactatgattaaaatgtatacgttagcatagaactgataataattgagctttagttacagcatttcctttctcctaacatctcccttacccagaaacaacttaaaacacttcaaattttttgagttagagatcacaaacatcaaggtatttgactcttattttccatcacttgctacttgagggggtcacactaaccaattctggttacatactttcctgctatggactctagaagaaaaactgcaaagaaacagaaaactaaccttcttaaacatatataaggaatcaagggtttccttaaactattacctgagagtcctatttttgccttctgtatagtaagcatgtcattctactcactattctgccggaatacatcttcacatttcaaactggattactttccaaatactggattacgttcatgcagtaaaaacaagaatagtgcatctattgaatatttttgcatttgcttattgcaatactagttaaaacaccagtttataatttttttatacattcagttgttcaacaaatgattcttttaatctgcctgaagtttcaagtcaacacgtcactggagaaaatgtatgaaactgtagcactaatttctgaaacgaaggattgaagttcctctttccaacttctttcagaccatcactactccacatgttcctgctcttgtcctggaattagccaccgaatactctcagttcgaatggtagcatacataataaaactaattaaaaagaataaggaaaatacaagcaaccagtccacactttttatcaaagtgctgggaagagggcctatttggtcggcttgagttaccaccacattcttcttggcttctatacctgtctgattaaaaatgaagattttcagtgtttccagtgttcgatctgtatgattaaatctggccattggtttagctccttgaaataataaaatattaggaacagctacggtgccaaacctggtagaaaggctgctgtgctgagatgcatccagtgccaaaaagtgaagagctggaaatgcccggggcagagagttaaagtgaggggccaaactggcagaaaagcggcaccacggggtgtaaaacaggactagagtacagtcactaccgtttgggttcagaaaatccataaggtcctgtgacatatttaaaattttcagagtgaaattttctaatcctgtaatgtttctctcctcacagttcacctttggggatttcagactttcagtgttattggagtcctctgtcggggctgcgtcagattccgccacttctggctctgtgtaatactcctcttctctgtcagggaagtgtgctccagcgccatccagagagaaaaggctctctcggacgttgcaccttgagtcctccgctcctccagcaccacaggtgacgccgctaggctctgaactcactttgtcctcagcttccccaggaatcacagacagcatcaccatgtgatcgccttgggtgtccagccccagcaccgcattggcctcttctgctgccctgtcctggcccatcgggtcatgcaggagctcctcctcacccaggtacacagcccccacctggagagggtgagcaggctgctcctctgaccataagcgaccactttcctctgcaacctccacgccgcggacgggaagtcccagcacccacagcaatacttgccaccagccgaggagccgcatgacgcggggcggtcgtcgaccggcagccgggaccattgcccaggccgagaggcaatcggcgcacggctacgcgagtcgtgctgccagccggag

SEQ ID NO: 15299 - RNA, 1249 nt, Homo sapiens
  source 1..1249: mol_type = other RNA
gctgggattacaggcatgagccactgcgcccagcctggaaacactattgacaagtgaggaggcctagtccattgagtatcagctagggctacaaacttccaaatcggtgaatcaggtccagagagggacaagtgccccagggttacacaatcatttgctgaagcagaggttgctgccatctttggcctcacccaactggaccacttccttgggcactgagtgacatagctccagcaggtctggattctgcagcttggtccttatcttctggctcagggtcagctccgggctcggcctgtgctgctgcagggcctccaggaccgagcgggccttctcaaagggggggatcttcagccggtacaggatctctgcccgcagatagttgccaatgccattgaagaacctctggtccaggagggcctcgcagatgggccggtcaaaggccttatccgctaggtttcgtagcacattctccctggaggaacacggtctgggtgcgtaagacccatccccaccctccatgggatggggagaggggctcagagaacctgtttctgagccctggaggttaaggctgcaatgagctgtgatggcgccactgtactctagcctaggcaacagagcgagaccctgaactgctggtactcctgcaagacacagggcccgcggcccggctgccactttcccccaaggtcccagcggccgaaccggcggatgtccacgaaacatagggcgagccgggggccaggcggggccgtgtaaaagcgcaggtgggcatggcgtggcagctcctcgcggggcaccagctgaaaagagccggacatgccgaagcggaagaccagggccagtggctcctgttggggctgggccccaggcagagggctcagtatcaggcgcagctccttgccgcgggctgaagctgagatgcggtaggcactgctctcaaagggcacctcagggttgcggctgacagaggacttctccacgcagccgccgaacaccagcgccctgcaggcctcattcacaaactggctggccaggtgcagctcggggccctcaggcatcctgagggagggtggcagagtcccggacaggtgcctggaaagcccagggcgctgggagctggggctgcagagggagcaggactctgccttgctgctaaccgcttccttccatgggcttccaccgcgtttagacgaaagtcccaatccttgcggggccgcggctgcagccttacttcttcccggct

SEQ ID NO: 15300 - RNA, 1585 nt, Homo sapiens
  source 1..1585: mol_type = other RNA
gctgggattacaggcatgagccactgcgcccagcctggaaacactattgacaagtgaggaggcctagtccattgagtatcagctagggctacaaacttccaaatcggtgaatcaggtccagagagggacaagtgccccagggttacacaatcatttgctgaagcagaggttgctgccatctttggcctcacccaactggaccacttccttgggcactgagtgacatagctccagcaggtctggattctgcagcttggtccttatcttctggctcagggtcagctccgggctcggcctgtgctgctgcagggcctccaggaccgagcgggccttctcaaagggggggatcttcagccggtacaggatctctgcccgcagatagttgccaatgccattgaagaacctctggtccaggagggcctcgcagatgggccggtcaaaggccttatccgctaggtttcgtagcacattctccctggaggaacacggtctgggtgcgtaagacccatccccaccctccatgggatggggagaggggctcagagaacctgtttctgagccctggaggttaaggctgcaatgagctgtgatggcgccactgtactctagcctaggcaacagagcgagaccctgaactgctggtactcctgcaagacacagggcccgcggcccggctgccactttcccccaaggtcccagcggccgaaccggcggatgtccacgaaacatagggcgagccgggggccaggcggggccgtgtaaaagcgcaggtgggcatggcgtggcagctcctcgcggggcaccagctgaaaagagccggacatgccgaagcggaagaccagggccagtggctcctgttggggctgggccccaggcagagggctcagtatcaggcgcagctccttgccgcgggctgaagctgagatgcggtaggcactgctctcaaagggcacctcagggttgcggctgacagaggacttctccacgcagccgccgaacaccagcgccctgcaggcctcattcacaaactggctggccaggtgcagctcggggccctcaggcatcctgagggagggtggcagagtcctccgccctccctgctttgccacttgcctctgtccccgggcggttcggaatcggaggcgaaggtgtgcctggctgggaggtggcggaagaacctgacttcccactgcctggcgccggcgagatgcgggggcaggtctgaggccccgggtcgccgctgtctctgcggttgggggaagtcacccagctagcgtgggacagggtcggcacccccagcaggaaacagcagcgacgagccagagcggagtcgcctgcagctgcgcgcaggacgtgcacaggtgcgcggtacgcacaggccctagggacccggtggggatcttaagcaccaacgaacagtcagacctaactcataaacaaacatcatcacggcctgccctgtcagaagcgcagccaagcaacaacaacaacaaaaaaaggcgaggaggtagacccacttgagatggttctgttgcggagagtctctgaaatcagaaagcgccagtccgcaaaaacgaggaaaccc

SEQ ID NO: 15301 - RNA, 1253 nt, Homo sapiens
  source 1..1253: mol_type = other RNA
gctgggattacaggcatgagccactgcgcccagcctggaaacactattgacaagtgaggaggcctagtccattgagtatcagctagggctacaaacttccaaatcggtgaatcaggtccagagagggacaagtgccccagggttacacaatcatttgctgaagcagaggttgctgccatctttggcctcacccaactggaccacttccttgggcactgagtgacatagctccagcaggtctggattctgcagcttggtccttatcttctggctcagggtcagctccgggctcggcctgtgctgctgcagggcctccaggaccgagcgggccttctcaaagggggggatcttcagccggtacaggatctctgcccgcagatagttgccaatgccattgaagaacctctggtccaggagggcctcgcagatgggccggtcaaaggccttatccgctaggtttcgtagcacattctccctggaggaacacggtctgggtgcgtaagacccatccccaccctccatgggatggggagaggggctcagagaacctgtttctgagccctggaggttaaggctgcaatgagctgtgatggcgccactgtactctagcctaggcaacagagcgagaccctgaactgctggtactcctgcaagacacagggcccgcggcccggctgccactttcccccaaggtcccagcggccgaaccggcggatgtccacgaaacatagggcgagccgggggccaggcggggccgtgtaaaagcgcaggtgggcatggcgtggcagctcctcgcggggcaccagctgaaaagagccggacatgccgaagcggaagaccagggccagtggctcctgttggggctgggccccaggcagagggctcagtatcaggcgcagctccttgccgcgggctgaagctgagatgcggtaggcactgctctcaaagggcacctcagggttgcggctgacagaggacttctccacgcagccgccgaacaccagcgccctgcaggcctcattcacaaactggctggccaggtgcagctcggggccctcaggcatcctgagggagggtggcagagtcctccgccctccctgctttgccacttgcctctgtccccgggcggttcggaatcggaggcgaaggtgtgccttaagtggaagggggcacttagcgacggcagacgcccgtaccttgccccctccacacctgggagccgcccctggcctggcacccacagggctcgtttt

SEQ ID NO: 15302 - RNA, 1226 nt, Homo sapiens
  source 1..1226: mol_type = other RNA
gctgggattacaggcatgagccactgcgcccagcctggaaacactattgacaagtgaggaggcctagtccattgagtatcagctagggctacaaacttccaaatcggtgaatcaggtccagagagggacaagtgccccagggttacacaatcatttgctgaagcagaggttgctgccatctttggcctcacccaactggaccacttccttgggcactgagtgacatagctccagcaggtctggattctgcagcttggtccttatcttctggctcagggtcagctccgggctcggcctgtgctgctgcagggcctccaggaccgagcgggccttctcaaagggggggatcttcagccggtacaggatctctgcccgcagatagttgccaatgccattgaagaacctctggtccaggagggcctcgcagatgggccggtcaaaggccttatccgctaggtttcgtagcacattctccctggaggaacacggtctgggtgcgtaagacccatccccaccctccatgggatggggagaggggctcagagaacctgtttctgagccctggaggttaaggctgcaatgagctgtgatggcgccactgtactctagcctaggcaacagagcgagaccctgaactgctggtactcctgcaagacacagggcccgcggcccggctgccactttcccccaaggtcccagcggccgaaccggcggatgtccacgaaacatagggcgagccgggggccaggcggggccgtgtaaaagcgcaggtgggcatggcgtggcagctcctcgcggggcaccagctgaaaagagccggacatgccgaagcggaagaccagggccagtggctcctgttggggctgggccccaggcagagggctcagtatcaggcgcagctccttgccgcgggctgaagctgagatgcggtaggcactgctctcaaagggcacctcagggttgcggctgacagaggacttctccacgcagccgccgaacaccagcgccctgcaggcctcattcacaaactggctggccaggtgcagctcggggccctcaggcatcctgagggagggtggcagagtcctctgtccccgggcggttcggaatcggaggcgaaggtgtgccttaagtggaagggggcacttagcgacggcagacgcccgtaccttgccccctccacacctgggagccgcccctggcctggcacccacagggctcgtttt

SEQ ID NO: 15303 - RNA, 1521 nt, Homo sapiens
  source 1..1521: mol_type = other RNA
gctgggattacaggcatgagccactgcgcccagcctggaaacactattgacaagtgaggaggcctagtccattgagtatcagctagggctacaaacttccaaatcggtgaatcaggtccagagagggacaagtgccccagggttacacaatcatttgctgaagcagaggttgctgccatctttggcctcacccaactggaccacttccttgggcactgagtgacatagctccagcaggtctggattctgcagcttggtccttatcttctggctcagggtcagctccgggctcggcctgtgctgctgcagggcctccaggaccgagcgggccttctcaaagggggggatcttcagccggtacaggatctctgcccgcagatagttgccaatgccattgaagaacctctggtccaggagggcctcgcagatgggccggtcaaaggccttatccgctaggtttcgtagcacattctccctggaggaacacggtctgggtgcgtaagacccatccccaccctccatgggatggggagaggggctcagagaacctgtttctgagccctggaggttaaggctgcaatgagctgtgatggcgccactgtactctagcctaggcaacagagcgagaccctgaactgctggtactcctgcaagacacagggcccgcggcccggctgccactttcccccaaggtcccagcggccgaaccggcggatgtccacgaaacatagggcgagccgggggccaggcggggccgtgtaaaagcgcaggtgggcatggcgtggcagctcctcgcggggcaccagctgaaaagagccggacatgccgaagcggaagaccagggccagtggctcctgttggggctgggccccaggcagagggctcagtatcaggcgcagctccttgccgcgggctgaagctgagatgcggtaggcactgctctcaaagggcacctcagggttgcggctgacagaggacttctccacgcagccgccgaacaccagcgccctgcaggcctcattcacaaactggctggccaggtgcagctcggggccctcaggcatcctgagggagggtggcagagtcctggctgggaggtggcggaagaacctgacttcccactgcctggcgccggcgagatgcgggggcaggtctgaggccccgggtcgccgctgtctctgcggttgggggaagtcacccagctagcgtgggacagggtcggcacccccagcaggaaacagcagcgacgagccagagcggagtcgcctgcagctgcgcgcaggacgtgcacaggtgcgcggtacgcacaggccctagggacccggtggggatcttaagcaccaacgaacagtcagacctaactcataaacaaacatcatcacggcctgccctgtcagaagcgcagccaagcaacaacaacaacaaaaaaaggcgaggaggtagacccacttgagatggttctgttgcggagagtctctgaaatcagaaagcgccagtccgcaaaaacgaggaaacccgacg

SEQ ID NO: 15304 - RNA, 1359 nt, Homo sapiens
  source 1..1359: mol_type = other RNA
gctgggattacaggcatgagccactgcgcccagcctgtacaattatttttaacagagaaatagagaagagtcctcaagaatatgaggaaacacatccttcaaaatagcttatgcaacattctctttgatagaccacctgttaggccaaaaacggagtcataaaaatttgttaaatttgacattttatgaattacatcctatgaccaaaatggaatgaaagtataaaatagaaaaaaaggctgggtgtagtggctcacgcctgtaatcccaacactttgggaggccaaggcaagtatactaaaaatccaattttttaataaaactttttataaaaacatgagtttttactaaaaactctcatggtggtgcatgcctgtagtctcagctactcgggaggctgacataggagaatcgctggaggcagaggttacgatgagccaagatggcgcctttgcactccaacctgggcaacaagagtgaaactccatctcaaaacaaaaaacaaaacaaaacaaaaaaactacaataaactttgaatagccaaagcaatcttgaggaaaaagaacaaagcagagagacattatattttataatttcagactatatttcaagaatatactaataaaaaaagatggaatgtgcagaaaattaacataaaaaccaatagaacagtgaccactactctcacacattttagacatgatgcaaaagagaactaaaaaaatagtttaacataaagtttctcaaaatcatgcagatatttgtgtgtcccccaaaacaatggaaatgcagtcagattgtgcagtcttttatatgccatgaagaggactctggctctcactgtgaacttgaaggaaaatcaatgaagggaaagtagaatccttagagaatttaaaagcctgggggtgtggctaccatactgtgtctcttcatattccagggatcttttccttgctccagacaggtgatcagatctggcttagagacatcaatacccaagaacaccaggtttctgaagttctctaacatcactttcctatacaaatcttgctgagcagtgtccaggcattgccactcctcctgagagaattctatgaccacatccctaaatgtcaacggccccttttcaaaataagagtactccagaagattcctctcagccccagggtatccacttgcccccttgacaggatacactccatacctcaggtcgtccatttctaggcttccagggtgtcccggcgtcttagctgtggattcccaatacctgcaggtcacaggaccagaggctgggcctctaggagcagaggacacagagcagtgaagacgagacccggagttccagcggcagccaaagac

SEQ ID NO: 15305 - RNA, 1360 nt, Homo sapiens
  source 1..1360: mol_type = other RNA
gctgggattacaggcatgagccactgcgcccagtcctattcgcttttattccctcaaggaaagctcctgggtttccgtcacgtgggctctgctccaggtgcaggacacagggaggaaaagagggggcttcttcccaccatggtgtggggagcagggtggggtgcagggttgagcagtacatacagaaggagggaggcagtgctgggatttgcacaggtgggcactcgaaagatgggtgtgggcagccaccaggatgggacagaaggagccgcaggaggtaagaccttcaggacagcagaaggggcagcgctgggccaggcaggctgaatcctggggtgggaggaaagctgagaaacacagctgcagaaggcaggcggcaggataagctgtgtggtctcacatccgtttggctgtgtgtgcattcgacggtcagtctgtgtctcagggaatttcctgaggcctcctttctgcttggtttccccaaaggagcttcctggatggacctgtcctcacaaaggccttcagctccttctaagtaaaggaacaggcaacctctgccttcccctgccacggattctctgattttcggattctctgtgagtccgttgatgtcccagaaagcgagtccagaagtgaccttcttcttgggaaattctccctcctgaagcccccggctgacttgaacacattgccaggtttgcgaaacaccgtgaataagagaactttttccaaaggatgtcgcacattcctgcctccaggaaagaccctgctatcctgaggaaaggagtatttcactgcattacagtttaaaatcttgaataattactgtttttccagttcttctttgaaattcaaagagagaggatagaaggaacaaatgcatggcaagtttgatttctgccacggaaggaatccaaacaggactactcacagctcatggcaagtttgatttctgccagggaaggaatctggacaggaaggaatccggacaggaaggaatccggacaggactgctcacaactgaactggagtgcctcctccatctccagtgtcacggcctctcctcttgctaaactttttgtttaaatgcaacactcttttctcatttgtcatggcatttgtcagaactgtgtttgcagatggaagacataaggttaaaagacgtccagatccattttagagacgattgaagtgaagcagtgagatcatctatcatctggcagaaattgggccaaaaccagacatcccccatccagccaagctgcgaagccttccagcacaaatgcgtctgaccacagctcacctgggattgtggccaggagccagttagccgggattggagagcaagcatgataaagtg

SEQ ID NO: 15306 - RNA, 4294 nt, Homo sapiens
  source 1..4294: mol_type = other RNA
gctgggattacaggcatgagccactgcgcccggcagagaaagtctcttttaaaactcatgtcttatccttctgggtgcctcaaactaggacctgttcagacataacagattcgtaccagtttattttggtgcaaaaactgggaaattcatacacaattttctcataatatgcaaaatatgtatttttccatgaacttcttgaagaccccttgtactaaaaagctgtattcaagaggatgtaaaaaggactgtagatactcaagtgccacttatttctgggatgcaaggatggttcaacatagtcaagcaaatcaatgtgatatgccacttgaacagaatgaaagatgaaaaccacatcatctcaatagatggagaaaaagtatttcacaaaattcaaaatccactcatcatagaaattctgaacaaaatagacagaaaaggaaatttacctcaacaatagaaaggccatccatgaaatgaccaacgagtagataacgaagcagggaacatggaatgattttcctgtaggatctcacatgatggaagaatgctctcaccccttctattcaataaatactggctgtcctagccagagcaatgaaatagcaaaagaaatcaaacccatccaaatcagaaagaaagaagtaaaattatatgtgtttgtagatgacatgatcttctgtgtagaaaatcacaaagactcaaccaaaatactactggaagtaataaacagattcagtgtatctgcacagtacaatatcagcaccaaaaattagctgaatttccatacattaacaataaacaattttaaaagaaaatttaaaaacacttccatttgctagagaacttaaagtaagaaatacttaggaataaaagcaaaaagatgagaagtttgtaacaataaacaattttaaaagaaaatttaaaaacacttccatttgctagagaacttaaagaaatagaaataaaagtaaaaaggtgagaagtttgtaccttgaaatctacaaatatacatcaatatgattaaaaacatatacagacatataacccatattgatggattggaaaaattaatattgttaaatgattatataacccaatgtgatttagattcaacacggtacccataaaaatccctatcagtttttgttaaagaacaaaaagcaaactgggaaaagtggctcatgtttgttggccagactgatctgaaactcctgacctcaagtgatctacccgccttggcctcccaaagtgctgggattacaggtgtgagacactgtacctggcccaatcctcttaacataaacactttaatgtcaattactgcttgatggtttgctctactcattgcatttggaacaattatctcaaaatgaattttctgatattctgcaaggagtgaagtcagactgaaaaccttgccacactgatgacatttgtaagatttccgtccagtgtgcattctctgatgtctaaggaggtgtgaacgtgaagtaaaggctttgccacaatcatcacacgtgaggtttctctcctgtatgaattctcctatgttttgcataggatgaagcttgactgaagaccttgcctcaatcatgacatttataaggtttgtctccagtatgagttcgccaatgaactgcaaggtatggacgatgtctgaaaaatttgccgattattacacttgtatgatctctcttccttatgggttctccaatgatttgcaatggttgtagcgttactgaagacttggtgacaatcattacattagtcaagtttccttcaccatggattgcctgatggtgagtaagtgttgactgctcattaaggctttgccagactcattacacttgtaaggtttctctccagtataaattctaggatgttgtgccaggtgtgagtcatgcccgaaagccttgtcacgaactcttacaattttatggtttctctgcagtatgatttattttatgtctttcaaggtttgacttgtgactgaaaactctgtgatattcttcacctttgtaagctttctctccagtatgaattctcctgtcttttgaggctcgatttgccactgtaaactttgtcacatgcttcacatttctaaggtttctctccactatgaagtctatgatgacgtggaaggtgtgcttgttgattaaaaattttgcaacgttcattacacttgtttctctccagtatgaattcttatgaattacaaggactgaattgtgacagaaggtcttgccacactcattgcacttgtttctttccagtatgaattgtatgatgatgtgcaagctttgcttttcaattaaaagctttgccacactcattaaacttgtaaggtttctctccagtatgaagtctatgatgacgtgcaaggtttgctttttgattaaaaaccttgccacattcattacacttgtaaggtttctctccagtatgaagtctatggtgacgtgcaaggtgtgctttttgattaaaaaccttgccacattcattacacttgtaaggtttatctccagtatgaagtctatgatgatgtgcaaggtgtgtttttcgattaaaaaccttgccacattcattacacttgtaaggtttctctccagtatgaagtctatgatgacatgcaaggtgtgttttccgattaaaacccttgccacattcattacacttgtaaggtttctctccagtatgaattgccgtatgaattacgagggctgaaattcgactgaacgtcttgccacactcattacacttgtaacgtttctctccaatatgaatagccttatgaattacaagggctgaatttcgactgaacgtcttgacacactcagtacacttgtagggtttctctccactatgaagtctatgatgacgtgcaaggtttgcctttttattaaaaaccttgccacattcattacacttgtaaggcttctctccggtatgaagtctacgatggcatttaagggttaactcctgactgaaggtcttgccacattcattacacttataaggtttctctcccgtatgaagtctatgatggcatgtaagggatgacttccgactaaaggtcttgccacactcattacacttgaaaggtttctctccagtatgaagtctacgatggcatgtaagggatgacgtctgactaaaggtcttgccacattcattacacttgtatggtttttctccagcatgaattctcctatgtcttttaaggtttgatttgaaactgaaagctttgtcacattcttcacatttgtaaggtttctctccagtatgaagtctacgatggcatgtaagggaatacgtctgactgaaagtcttgccacactcattacacctgtaaggtttctccccagtgtgacatctacgatggcacactaggtttcgcttccgattaaagaccttgccacatacatcacatttatattgtttctctcctaaatggattatttgatgtttccttaagagtgagctataattaaaggctttgccactctcattacattggaaagacttttctctcatgtgtacctcctgtttttgtgtgagtaacgaagaattccggaaattattcccatagttattagaaatatgggttttgggcctacaagaaattctttgggatgttgaaattgaggaagcatcgttgatagacttctccacttgattaccaattttcccttgggtctgaaacatgtggagttcaggcagatgcgaatgaaagcttgatccaagctgatctttaataggcttgtttccagcatgcctttgatcatatcggtctgcactaccagtcaactttttgatttctgtcatgggtgcttcatggctatttctttcatcttcttgccactgaaactctaagttatgaatatctttatcaatttcctgaaagcgaaagtctccagtgtgatgactttcatgtctttgcaatgtccctgtgtggatcacttctctattgccttgtgctgttgatgagaactccttcatcatgcatttggaagagatatccagggagaccaggttcctataattctccagcatcacgtccctgtatagagtcctctgagcagggtccaggcatttccactcctcctgagagaattctatggccacatccctgaatgtcaatagaccctgaggaagagccatccctgactcctttgctttcctcttcctcttccaggtttcttcctcacataccaagagtctttagaagtcaatcgcgctgccgtgggaccgtcactccacgcgatccgcttccgggttttcgcgaatctgc

SEQ ID NO: 15307 - RNA, 1733 nt, Homo sapiens
  source 1..1733: mol_type = other RNA
gctgggattacaggcatgagccactgcgcccggccaaaaaacaactctttaaaaatgtaccttagagcaacatgcaaagcttccctgctcagcaatcccaggttggggccccctgtcttcctatcgtcctacccgtcacaaccaccactgcaggcttctgatgctctgttttcctcctctgtctcagttcagttgctctgagttagagaggagctctctgggactggagctgactgcgccctggcccatttcctcactaccatcctcaagctcagatgctgacaggaaaatactgcctatgcctgaaggggcatcccttagcaggcggcccagttccttctcataacatttggctgcttgcagcagatctccattctgcttatgaattaatccttgaagataccaataatttggtgcattttgtggaagcagattttcagatacattctgtggttggtctttgatctcttccttgtcagttgattttttgcttatggacaaaccctctaaaccatgttgcacagcagtgtcttcagacttcccattatatttctgaaggttgcagtagcgctgatgggattgttgcttttcagcatcagggacttccttattgaatggtgtctgataacattccgtctccaggaactcagcgagatcggagtatgcattcagaggattcagtcccttctcaagagctttattcgaatagtccatagcatattgctttagtgcttcaatcatctctttatttccactagcttcagattctcctgtattctgcatttgtcttacttttgccttgtagcagcacccaatctggtgatagaggtagccattgtttggtgtggattccaacacccgttgaaacagttcaatagctttgtctaggtcaccttttcttctgtaaaatttggctgcactgcggaggacatctgtttggcaaggagacttttccaaggcttcttcaacaaactgctctccttcagcttctttattcatcttctgcagtttcaggcccaagagaaccttgacgtattggttatcaggactcagctcaatggcctgcttcaaaacatcagtagagaactgtttctctgggtgattatccagatggtacatcgcaattgccagtccagaggagaattctgggttgttgggcttttcttccagagccttctcaaaacacaccttcgccctttcatttcttccacacttcagttgtgtccacccttcctcacagtcaagttcagaatactcaatactgtatggatttgaaaatttcttgcaggtttgtttcaccttatctacataaatctgagcatctgagagtctgcccaagtgatagtagacccaggcgtagtttccccaagtgactagacttctgatttctgcttggtcagcatgttcttgctggattaactcttcagcttgccgtaagcattccagggctgcctcgttgttaccatctaggtgttttatgtaggccaacaagttgtacattgtagctttgaactcagtgtttaaaaattcaatctggttacacactctatcttctagatcccttgagacactgtcttccttgaataagttccaggtgaaatggcatttcagctgtggaaggattttctccagggaattcttggtgacctcactcatgactgccctctgtgtctctgctgttccgaaaagctggtgaccaggctgatttgttcttcagaagtcttcctgtctgc

SEQ ID NO: 15308 - RNA, 1750 nt, Homo sapiens
  source 1..1750: mol_type = other RNA
gctgggattacaggcatgagccactgcgcccggccaaaaaacaactctttaaaaatgtaccttagagcaacatgcaaagcttccctgctcagcaatcccaggttggggccccctgtcttcctatcgtcctacccgtcacaaccaccactgcaggcttctgatgctctgttttcctcctctgtctcagttcagttgctctgagttagagaggagctctctgggactggagctgactgcgccctggcccatttcctcactaccatcctcaagctcagatgctgacaggaaaatactgcctatgcctgaaggggcatcccttagcaggcggcccagttccttctcataacatttggctgcttgcagcagatctccattctgcttatgaattaatccttgaagataccaataatttggtgcattttgtggaagcagattttcagatacattctgtggttggtctttgatctcttccttgtcagttgattttttgcttatggacaaaccctctaaaccatgttgcacagcagtgtcttcagacttcccattatatttctgaaggttgcagtagcgctgatgggattgttgcttttcagcatcagggacttccttattgaatggtgtctgataacattccgtctccaggaactcagcgagatcggagtatgcattcagaggattcagtcccttctcaagagctttattcgaatagtccatagcatattgctttagtgcttcaatcatctctttatttccactagcttcagattctcctgtattctgcatttgtcttacttttgccttgtagcagcacccaatctggtgatagaggtagccattgtttggtgtggattccaacacccgttgaaacagttcaatagctttgtctaggtcaccttttcttctgtaaaatttggctgcactgcggaggacatctgtttggcaaggagacttttccaaggcttcttcaacaaactgctctccttcagcttctttattcatcttctgcagtttcaggcccaagagaaccttgacgtattggttatcaggactcagctcaatggcctgcttcaaaacatcagtagagaactgtttctctgggtgattatccagatggtacatcgcaattgccagtccagaggagaattctgggttgttgggcttttcttccagagccttctcaaaacacaccttcgccctttcatttcttccacacttcagttgtgtccacccttcctcacagtcaagttcagaatactcaatactgtatggatttgaaaatttcttgcaggtttgtttcaccttatctacataaatctgagcatctgagagtctgcccaagtgatagtagacccaggcgtagtttccccaagtgactagacttctgatttctgcttggtcagcatgttcttgctggattaactcttcagcttgccgtaagcattccagggctgcctcgttgttaccatctaggtgttttatgtaggccaacaagttgtacattgtagctttgaactcagtgtttaaaaattcaatctggttacacactctatcttctagatcccttgagacactgtcttccttgaataagttccaggtgaaatggcatttcagctgtggaaggattttctccagggaattcttggtgacctcactcatgatggctgtttccctgcagttctgaaaagctggggtcccggttgattttgtttttagcttactgattccaagcaaatgctgaagaggtttccac

SEQ ID NO: 15309 - RNA, 1851 nt, Homo sapiens
  source 1..1851: mol_type = other RNA
gctgggattacaggcatgagccactgcgcccggccaaaaaacaactctttaaaaatgtaccttagagcaacatgcaaagcttccctgctcagcaatcccaggttggggccccctgtcttcctatcgtcctacccgtcacaaccaccactgcaggcttctgatgctctgttttcctcctctgtctcagttcagttgctctgagttagagaggagctctctgggactggagctgactgcgccctggcccatttcctcactaccatcctcaagctcagatgctgacaggaaaatactgcctatgcctgaaggggcatcccttagcaggcggcccagttccttctcataacatttggctgcttgcagcagatctccattctgcttatgaattaatccttgaagataccaataatttggtgcattttgtggaagcagattttcagatacattctgtggttggtctttgatctcttccttgtcagttgattttttgcttatggacaaaccctctaaaccatgttgcacagcagtgtcttcagacttcccattatatttctgaaggttgcagtagcgctgatgggattgttgcttttcagcatcagggacttccttattgaatggtgtctgataacattccgtctccaggaactcagcgagatcggagtatgcattcagaggattcagtcccttctcaagagctttattcgaatagtccatagcatattgctttagtgcttcaatcatctctttatttccactagcttcagattctcctgtattctgcatttgtcttacttttgccttgtagcagcacccaatctggtgatagaggtagccattgtttggtgtggattccaacacccgttgaaacagttcaatagctttgtctaggtcaccttttcttctgtaaaatttggctgcactgcggaggacatctgtttggcaaggagacttttccaaggcttcttcaacaaactgctctccttcagcttctttattcatcttctgcagtttcaggcccaagagaaccttgacgtattggttatcaggactcagctcaatggcctgcttcaaaacatcagtagagaactgtttctctgggtgattatccagatggtacatcgcaattgccagtccagaggagaattctgggttgttgggcttttcttccagagccttctcaaaacacaccttcgccctttcatttcttccacacttcagttgtgtccacccttcctcacagtcaagttcagaatactcaatactgtatggatttgaaaatttcttgcaggtttgtttcaccttatctacataaatctgagcatctgagagtctgcccaagtgatagtagacccaggcgtagtttccccaagtgactagacttctgatttctgcttggtcagcatgttcttgctggattaactcttcagcttgccgtaagcattccagggctgcctcgttgttaccatctaggtgttttatgtaggccaacaagttgtacattgtagctttgaactcagtgtttaaaaattcaatctggttacacactctatcttctagatcccttgagacactgtcttccttgaataagttccaggtgaaatggcatttcagctgtggaaggattttctccagggaattcttggtgacctcactgtagtcctcgccattcgggaggctgagacaggaggatcacttgagcccaggaggcaaaagttgtagtgagctgagatcacaccattacactccagccagggtgatagagtgggaccctcatgactgccctctgtgtctctgctgttccgaaaagctggtgaccaggctgatttgttcttcagaagtcttcctgtctgc

SEQ ID NO: 15310 - RNA, 1872 nt, Homo sapiens
  source 1..1872: mol_type = other RNA
gctgggattacaggcatgagccactgcgcccggccaaaaaacaactctttaaaaatgtaccttagagcaacatgcaaagcttccctgctcagcaatcccaggttggggccccctgtcttcctatcgtcctacccgtcacaaccaccactgcaggcttctgatgctctgttttcctcctctgtctcagttcagttgctctgagttagagaggagctctctgggactggagctgactgcgccctggcccatttcctcactaccatcctcaagctcagatgctgacaggaaaatactgcctatgcctgaaggggcatcccttagcaggcggcccagttccttctcataacatttggctgcttgcagcagatctccattctgcttatgaattaatccttgaagataccaataatttggtgcattttgtggaagcagattttcagatacattctgtggttggtctttgatctcttccttgtcagttgattttttgcttatggacaaaccctctaaaccatgttgcacagcagtgtcttcagacttcccattatatttctgaaggttgcagtagcgctgatgggattgttgcttttcagcatcagggacttccttattgaatggtgtctgataacattccgtctccaggaactcagcgagatcggagtatgcattcagaggattcagtcccttctcaagagctttattcgaatagtccatagcatattgctttagtgcttcaatcatctctttatttccactagcttcagattctcctgtattctgcatttgtcttacttttgccttgtagcagcacccaatctggtgatagaggtagccattgtttggtgtggattccaacacccgttgaaacagttcaatagctttgtctaggtcaccttttcttctgtaaaatttggctgcactgcggaggacatctgtttggcaaggagacttttccaaggcttcttcaacaaactgctctccttcagcttctttattcatcttctgcagtttcaggcccaagagaaccttgacgtattggttatcaggactcagctcaatggcctgcttcaaaacatcagtagagaactgtttctctgggtgattatccagatggtacatcgcaattgccagtccagaggagaattctgggttgttgggcttttcttccagagccttctcaaaacacaccttcgccctttcatttcttccacacttcagttgtgtccacccttcctcacagtcaagttcagaatactcaatactgtatggatttgaaaatttcttgcaggtttgtttcaccttatctacataaatctgagcatctgagagtctgcccaagtgatagtagacccaggcgtagtttccccaagtgactagacttctgatttctgcttggtcagcatgttcttgctggattaactcttcagcttgccgtaagcattccagggctgcctcgttgttaccatctaggtgttttatgtaggccaacaagttgtacattgtagctttgaactcagtgtttaaaaattcaatctggttacacactctatcttctagatcccttgagacactgtcttccttgaataagttccaggtgaaatggcatttcagctgtggaaggattttctccagggaattcttggtgacctcactgtagtcctcgccattcgggaggctgagacaggaggatcacttgagcccaggaggcaaaagttgtagtgagctgagatcacaccattacactccagccagggtgatagagtgggaccctgcctcatgatggctgtttccctgcagttctgaaaagctggggtcccggttgattttgtttttagcttactgattccaagcaaatgctgaagaggtttccac

SEQ ID NO: 15311 - RNA, 312 nt, Homo sapiens
  source 1..312: mol_type = other RNA
gctgggattacaggcatgagccactgcgcccggccaataagctgattcttaatggagatgacaggaactattctgcttgaccagtagagtgctttccaagatcttgatcatcatttcactggtagattattgcagaaaccctcatgctcctaaacgaccataagaaactgagctcaaatttgaaggcatcacttgtatcctgtgaaagagaaaccaaagaatgaccaaacccctcagaaattatgtagctcctggctgatcgtcacctgctgattcctctaaccatgcttggggcaaaggtaatgcagctgt

SEQ ID NO: 15312 - RNA, 844 nt, Homo sapiens
  source 1..844: mol_type = other RNA
gctgggattacaggcatgagccactgcgcccggccaataagctgattcttaatggagatgacaggaactattctgcttgaccagtagagtgctttccaagatcttgatcatcatttcactggtagattattgcagaaaccctcatgctcctaaacgaccataagaaactgagctcaaatttgaaggcatcacttgtatcctgtgaaagagaaaccaaagaatgaccaaacccctcagaaattatgtagctcctggctgatcgtcacctgctgattcctctaaccatgcttggggcaaaggtaatgcagctgtaaaactgactgtgaattctacaaggacttattgagcagacatgtctgagcaaaggaccagattgcacaatggttggcatcaggtgccactggggctaagtgcatggtcactgttcctctcttctatagtgatagattatctctgatgctggcttgctgcctcgaacaaatgccctgagtgaagtgccagataagagaagggatgagtccacctccatttataaaatctaaactaactccgagcccctatggctcactggacagccatcggtaagtggtgtctagaagggattgctgtatttggctataggtagacgaggggacatttgagtctctgaccattggttaaaagggcaatcttggaaacaacagacactggggactccaaatgtggaaaggaaaggattggagcaaaggttgaaaaactacctattgcatacgaggttcactaactacatgatggattcaactgaagcccaaacctcagtgttacgcaatatacccatataacaaatctgcatatgtacccccaa

SEQ ID NO: 15313 - RNA, 727 nt, Homo sapiens
  source 1..727: mol_type = other RNA
gctgggattacaggcatgagccactgcgcccggccaataagctgattcttaatggagatgacaggaactattctgcttgaccagtagagtgctttccaagatcttgatcatcatttcactggtagattattgcagaaaccctcatgctcctgctgattcctctaaccatgcttggggcaaaggtaatgcagctgtaaaactgactgtgaattctacaaggacttattgagcagacatgtctgagcaaaggaccagattgcacaatggttggcatcaggtgccactggggctaagtgcatggtcactgttcctctcttctatagtgatagattatctctgatgctggcttgctgcctcgaacaaatgccctgagtgaagtgccagataagagaagggatgagtccacctccatttataaaatctaaactaactccgagcccctatggctcactggacagccatcggtaagtggtgtctagaagggattgctgtatttggctataggtagacgaggggacatttgagtctctgaccattggttaaaagggcaatcttggaaacaacagacactggggactccaaatgtggaaaggaaaggattggagcaaaggttgaaaaactacctattgcatacgaggttcactaactacatgatggattcaactgaagcccaaacctcagtgttacgcaatatacccatataacaaatctgcatatgtacccccaa

SEQ ID NO: 15314 - RNA, 12850 nt, Homo sapiens
  source 1..12850: mol_type = other RNA
gctgggattacaggcatgagccactgcgcccggccaatctgaaagttttctatgcacaaatctagtgtgcctctgaagtctttcaagtcaacctttttttggccccatactatgttgctaccgacatactataatccagttctgagaaaatcaggactgacagactttaaaaatgacactgaaaagcgacagacaggtttgaacctggcttaaccacataaaagttgaacaaactctctgagctctggcttccttcattataaaatgggcaaattcttgccttgcctttttcacaaagttatcatcaagatgaaataagaaaaataaaaagtatttctaaaagtgcttgtgtgtttgcacatgtaaaagagaaaaagactacttcagaccttctgtaaaaattcaaccaggttcagcgaactaatgatggcaggatctggagtaagctttgcatttcatgcctcagttttctcacttgtaaagcttactcttcctggcaggctcagggaagtaaatactgaaaccagtaaagcatttggtactgagcagttaagaaaattgggacgaggcctcagggggttttggataatatgaaaactctatttccgaatccttcctaaaaccagacctccatgtaccaaccaataaaactttcactgcagagactataggatccaaatgtctctgtctcttctttccttgtccccgtgtgaacagcaagcctggctcattctcagtccccaggtagttatcctgagcctgcctttctcagcagcaagggcaagggcagagaggtggggtggggaagggggaaggtaattaaaatggccacccattcagaagaaaattgagtccgtggaggggaaagggcagggagagggagcaaaacccttagtgctgaagcaccaggaagaaaggcaagacacaaaagagggaagaaggcagtaatttagtggttgtcttgacgaccagagtccctattgttcatgggggctttacctcacagggagatctccctgttctgctctgcacatagaactcccaccacaggaaaggaggatgggaagggaagggttgcaggaggcagaagtgataagtaattatgtgctcgcagaaggggctgacctccaaatttctgcaaatattacggataacagatttagagtgtgctcagccatgatttggaagaaaattattagggatttatttaaatcagcagacatgggaggacttcaaattatgctgtgaaaatggctacaggaggctggaaaagaccagccttgaggagaataaagaatacatatatgagaagcagatgcccaagataaacaaagagaaaaaacactgagaggggtgtagaggagaaggaaaagtgactatcattaacaccatcaccttggtgtagaagagctacccaaaagtatttccagttccctgtctacaggctgaaatgtaaaacctttccaagtagaaggccatctatcccgttatgaaggacgtagggacaccgaagtggcaactccagaatctccacagaataggaactttgggagcactgactatgggtagaaaacacagaggagtaataaataaaactggaaaaacaacaaaaaggaaacctgggggagagaggaggcaggtgttgaggaacttaccttgatgctgcatttgcacaccagcctccctcccaggaaggctgaatcctctccgagaaatctttcggggccagcattatattagagctaaagtatatttcccaccaatttacccaactccctccctgctccagtaccaaatagctctacttctccaaagggcacttggagaagcctgcaaggacagaggtaaagatcaaaagtaagcaataacatatggttgcttctccaaaaccaagttaatgggggagagccaaacggtctccatccatggccgaaagcaatagggaatgtccttgattatgtaacaggttgataagattcctaacatcggggctattcagcactgacaatctccatcttagtgaatacataatgtataagattttaggatcacaggagaccctgaatataggtccaagtagtttatacagaatattaacaaaattcttgcaattcagatgtctagctggtctcatcaccacagactctgttctgctcactctgttctgaatgaatcagctccagcactgaatttttaacgggtgggatccactcaaaggggcaacttctggtcatccacaccactcagagaagcaagcatatgctgaagacgcattagagcagaaggaagaagggtgaaagatcaaagaaacagggcttatctaaaagtcactggcactaaggagtaggcagataagtggcctctaaaccgtagagcaagccagggaatggcttcaatatactgtatcaacatcacggcaggggacctataactgcaaaacaaacaggtcttcctcaaaggacagtgaatggtattgtttaacctgcagcgccacctggtgcccatagagagaattcctgtgcccacgccatgcagcagcagtttggtaggctttttgtcacctatttgaaacaataaaagcaacacacattcagaaagaagctggctaaaaatattccaggttgctttttatttgaaagtagaatgcccctcctcctgttttaaaaatgtcttagtgtctagaatattatttagcctaaaccagtctaaatgacacctatctcacaagatctagctgttataccttcctctataaagcctctctaacatttacctctaaattatctcttatccccccaaagaacttcatgcactaggctatgatttctatttcgacagtaacagacaaaggaagttaagtggtttgttctaagtcacatagcctcaaagcaagatctgatttcagatctgacttcaaagtccaagttcttgctttccatgtggaaggaaagaggtggagaaagtacaacagcaggagatgcttccagagagggcaggctcggtggggcttcatactgggaggcccaggttgtggaggggcgctgcactctttggaaaggagagagccattagaatgggagatggcctgaagggcccccaaacctctttgcttaggccgtaccatggctctgggaatcagaattccccaattaactgaagatctgggtatgccctgtgtggagggaatgaaagactcagtttccattttgcttctggtcccccagcactgttgaggaaaccctaagattcttaatagtgataagcagagggactgcctccagtagaatgacgtgtgatcttctgtgttcatttatttgacacaaatttactaggtgccttctatgcatggggctgggtgttgaagatataatggtaaataagacgcagtccctgccctcaggatgctgacatacattctaaagctgtcatcaaaatgtcaaaatcttaggttcctgtttgcagtcacagatgggcaagagatgccaagaacctgacttggaaaaaaaggctctgaggtttaaatacctcatgatattctgttttttgttaacttttacaatgagcaattttgtacctctatttgagtatatgagacttcaagagcacacacacacagaaatgcaaatgcaatgctcaggcacacggctgtcagctgccatccacctgctacaatctcaaagatatattccagtagagactgtcactatgtgacaggaaagccatgatgtcttcatcctaagatgggtgtagaataagtgatacccaagaaatatgacaggcagaccactcatatgacaggggaaactgctagggcccatcctggcccagtctatagaagtcaagagcttccctttggcatggcctaatggaagaggcctgggacaagcagtactccttcccagggagccacagtacaatctgagcaaagccatcaatgagaaaaattaatttcagcacctctaaaaacagcccaagccaatgactggagagccagaaaataagcgagaattctgaagactgagcttgagttaattttgtatgtgggggtcttgcaaaagtatgcgtatttctagaaaagctgtgcataggaagagatggggtataagacatagccaggcatcagagctgaactggaagaaaaagttacacagcaaaggaaaaaactgtaatctatgcttcctgagaaactctgagtcttaacgttgataatcttttcctgattgtgaatagcatataaatagagatagctaagagacaatctctggctcagaagtgctttaaaaataaaatcagaatatgcagacaaaaataatttatatgctaccatcagatgcgtgtgtccctgagaccagctggatggaaagcaagagaggctagatgggaatacggcaagggaactttcaggtgaacccagttctagtggccactgctttgtgggaaagcttgcatggaggggaagcatggcagagcagtgggaaacacatgagctctgaggccaggatgacttaagtggaatcttaaggtgtggttgttacgacttttatgattttgggaacgttattttatctgaatgtaattttcttcacttatgaaatgtagaactacatgtctatctcatagaattgaacattaatataaacagtacatagctgctttcctggtattaatattgtaataagcgtcagttcctttcccattgcaattactcgtgcacttttggtggcagacctggaggttctcttaagaaataaccaatgtcacaaagaactgttatccacctgctagttagacatgcccaccaagaaagaggcccttgaagtagagttccacagaaagcgccttgattctggagcgttctaagagaacagtggaagcaagagggttcatggtcaacctttcccaactgtccttaggggaggtggacgttgcgccttgcagcacagcactctccagtgctcccagactctgccgcagctctcctgacctttcctaggagatggtttagagagagacatcttctctaagaaagtgattccaaggtctggtgtaaggtctagagcttgccatcaagtttctcctgggtgccctgcttgttggactccttaaacctgcacaccctttcttttcttcttcctctctggatacttcctaactttacacacttcacgctcccctctgccagaacctttccccctggctttctgccaagccattccattcccacatgcccccaacactcacacacacacactctgtctctatcttacacacacacacacagacacacacacacacactccctttttaactgagaaatcctgacgcagatgccaggaatgtgtctgctgcccttttgacacaggtctgatgccatcgttggggccatggggagggcagcgccgcggacgtggcattcacgcattctgctgctggcatggttcctatttttatcgtggcattgctctgggtgtccaggcagggcgccggtccagcttctcattccttcactttccatcaggactccacaccaatcctaccccttaccttggctggatcttcctgccccaaaccccctaccatcaatgcagcacagtgtatctctcctctttccctccaacccagtctaactctgagtacttgcccagtttgctaaatctgattctgatgtttgcagagatattttcaagtttcttctgttttcgggcatgagcagagtttgcacaagccggatttgctccttggctcagagtgctacccgctctccccttcccctccctttgtctctcattccaaataaggagtgcttcttgttacataattggatgttcccagcacagaagctgacacatgaggttaggcgcacatgcatgcaagacttccctttgacttaacaatgccttttttgggcatctaacttctcttcagctcccctcccacttctctccacatcatcaacaatcaacggagatttataagcctggctcagatcagagctcttccaactttggcttagaaggaggggttatgaggtcgaacttactctgttttttttttttcctttgcaggatagagagtgtgcttataatttgacagaagtctatggcgtccaaggcagtaatgtacacaggtcttttaaagttgcaagatgggtatacaaagttggaagcagaggaataaacttgcctgcttggggataataatactggaggttggaacatgaggacattttaaggaggagatgcactcaaatctggtgactacagcatccctgatggtcaaactgcagtgagttctaaataactagagaagtggcagtaccacgtgtggcaccaacaccaactatcctgctcttttaagcacggaacttaaaggaagagaacccaagtaccctgcaaaagcatatggctcagctacccgtggtttcagggaggacaaacatgtagcctcctaggcagcagtcatggggatgggaggcaacgggacctcatatcatgcctcttgtgggagatgcagggggtacagtggagaggtgctgcagctctggagatgtcaagtttccagcatattggcttaccaaagcaaataaagctgaagcatgcagcaatgcatacaccactttttaaaattaaaacctgcaactgtcccagggatagtaacatgggctgtctttagactgcagcactgcccttaggttagctgcaagtgtgtagatacggagatgcagtttggattctacaaactgcctgataatctccagtacttggagacagagatttttgggttggcttttatcctgctgaattgcagggcaaagatctgatcctgaaatttagacaatcatcacagctataaatcagaaaaacctgggttcaaattctgcttgtgatatttattaaccctgtgattttgactagataacccacattctttgtaaaccttagtttccttgtctttaaaatgagggtcatagtaccgctttcgcaggacttggaggaattaaatggtattaagttggtgcaaaagtaactgtggcttttgaacagcatgtgcatacagtgttcagtacagtatttgcactaagtcaactctcgataaacatttgctggacagcaaatgtgctgatgctgacgagattatcaacgtttacactctgaatgctaaaatgtgttagctccatgtctataatgcacagggtgcttccaggtatgagaccatgggccaccagtgccagatctttggaagctctagtggaagaaccggttctttctttagatatcatgacttctagcttcctatcttaaggaggcttcaggaaaactgtgaaaccagctataaggtacttcagaagagggccaaaaatgtcattaaaaagatgggaaaaatgatttgtagggatacatgaatggcctcaaacagagaagtatgagattcttcatttaattctagtctgtggaagcttgggtgaggagactgctaaccagatgtggtcctattttcattgcagctaatacaaaaccaaatgggctaaggataaagttgtattcttagatataagaacttgttgacaggaagggatatgaggtaactgaacatgtataaaacatcttcacctggaaatatgtacaatgaaccaaagataacaggccatagttacaacaagtttttcaaaagtaactagccgcaaaatgctgttcttgcccaatattcacagtggcttcattcaaattcaccaaatatattcagagttttcccacttttcccatcacaatagtgatgcttttccataaaacagaataagacaaaaccaaaaaacaaaaagtcagaatgtgaaaagaggagaaagtctagggaaattcagctgtaagccctctccctcatttcctttatggcatgagctacatttgggttttgctagtctgcattcaccagactttacccagctcactggagttgtggttgtagttggggagtgtcagggacaggaatggaaaggtgaggaacttgcctgggcaacatagtgagaccccatctcaaccaaaaaatttaaaaaattagccaagcacggtggtgtgtgcctgtagtcctagctacctgggaggctgaggtgggaggatggcttgagcccaggaggttacagtgagctatgattgcagtgccactgcactccagcctgggcgacagaatgaaatcccatctcactgatatttcatatattgacattttatcctcaatatatgaaaaatgaaaaagaaagaagtctcacagcctctgctctgaactctaaaatgagccctgtcttttccatgtctgccacgcagctggagcttgcttcgctcgtatttaacttttctgccttagatctcccagggccccggccacatgaaaaagtacttctgtgatcattctctaactcccagaatataggtatttctcctttatctggactagcccaaacccttgagcactctgagttattcaaacttcaggtcaactttttcctaccccttttatataaggatctcaatcttttttgaatttctcctaactcatctatacttttatcctcatactgaataatttctcgtgttctgaaaccaatctgtcatgtaaatgacctcaaggagaaggggtcatattagatcacacactagctagttttgggatcttctcattttgtttttttaaaccacttagaagattagcaaagggaagtccaaaaaaagaagaagagaaatgaaggcctaattagtgacatccagaggtgacagaataaaactaaagagactatactttcaagtgtaaaggtactgggaagggaaatgtttatttctttattcaatatttaatgagtacctactatgtccaggccctgtataagctgctggggagacaaagctagttccggtccttaaagaactaatagtctacacagcatttctcaagcttggtaacactgatattttgggcaggataattcacgttgtttggcatggtggactgtcctgtgtagctgcaggatgtttagcagcatccttggcctacatccactagatgccagtaggcatcccacatctccttcccagttgtgacaacaaaaaatatctccagataatggcaagtgtcccctgggggacaaaagtgtaccccagttgacaaccactagtgtaggaaaagcagatcatttatataaacacactgtgacaagtattattatcaaaactttgcaagttagagaagaggactccttaattctcggggaaagagagcagatgctacagaaggtttcacagaataaatgacattttatgcttaatatatgaaaaatgttttgcagtaggccaagcagacaagaagaggaaaagttaggaacacatggaaggaacagggaaataacaggtagagaaagaccattcgaaggcagatacaggaagatgagcaaaggcctgggggtaaaagaccacagaatattcaggcaatgatggacgtttacacggtggaaaatgaaaaataagactgaaaccagatcatgccaagtaagaaaggaggtggaattttaatataaagaaataaatgcatattttaaacagagtggagccccttttcaaacaaagcgttacctagagccccagtatattaaactgatcaaagtgtaacttctgtggttgggtcatggtccactcagttttccctgagcttctaagttggcttcagaagcacttctgcagaaccctagaactctttgaactagggtcccaaagataagacgaagaaacttttgcatgttttcggtacatagccatttccactgttctgttagtagcaagaggagcagatccagggctgtgtcagctaactctgtctctgttcctggatcgctgttgctggggtcttgggctggcacggctgcatctgacacgcaactgtccacacgtcctttgggaggttgttcaggatctttttctggggcttttgttggctgcatttccagtaactttgtctgtttttcaataaaagattccatcgcagacatggatagagtctcagactccacattgccttcctggagacaataaagaatcttgtcttgtgcttcagtcacacttagtgctggagaaattttactggatgagaacctcagcctagacttgctagccttcttgccttctgtctggggcttgctttcggtctcggcctcactcagctcctctgtggggctctggggttcagagcgaggaaacgctgtcttcaaggtgtccacaatggcactcaccaccatcttgtctattctagagaccataaatggtttcttgacaaaggcaatacgagcatctgtgttcagagcaaggaactcctgcacctcctcactgttagcgatctccggaatggcacagagttgctttaggaatgattctaggaggctcttacgggcttctactctgtcactgtccatgtttcccaatggaagatctggaaagagctttttaggacccttcacatttttgatgaactttcgtagatctggtttctcctccagacgggtctgcagattcaagaactcccgatagcgacgattcacagtgtggtaggccagctgctgcaggccgctgctgttttcaccgtcaagggctgtctcgtacttcacagtatagagtgtgtatgggtggaatccagtgccactgtgctctcgggctgtaatggtgccagtgatacgaaggttctggatgataactggaccatcgggactgcttaggggctcaaagctgaaggtggctgagctgagaggaccaggtggagaggaggaaagcagaactggtggcagagtaggatcaagggagctcacatcattggtgagatccttctctaagcatgacggccgtgaggggcaggtcttttctggcccctccagcaaagctgtaacagaggcggtaacatctccttgttctatctccttgtctgctgtgtcaatatggatctctgggcaggaattcagtgtggagaccggcaggcctgtctctgtttctgtccctggaccctcctcagcctctgctccttcagatgcctcaccatctttgggttccagagcctgggaactctctagggcacacagggcatcctgaatcctgtcagagagaaagctgcctggagtcatgagcatgatggtttctttgcccagttcagacagcggagactccagctctgagtcttcacataagaacaggggacctcgaacatttggctgtaggaaatgagatgagttgtttcctacttttctttcttcacacatcccacccaaatctccctctacagcttcgtggccttcttcaacctctggagaggggcctgcagaaccctctggctcactgtaacttaggaatactggggctgctactggagaagctctcccttctggaagctgctctacctcagcaatcagtggcagagatgtcggcactgagggctgttcgggggcactggctgggcagggtgctggatctctggccttggaaaagatacccacgagtacaaggtggatccagtcaggatctgacagcctgctgatcagtggtaagattacattgcatgtgatgagttcgaccactacatggcgtccggtacgagtctccaagtggggcttgggcaccagcccttgaagcaacaaattcacaacgccacgcgtataggtgacttcagcactggggctgtgcacagcaggatgtggggcagtcgcccggcagtaagcctcccagaggtgggaaggctcaactggaccattcttccctgcagtggcctcctttgcctgaatgtagctctgcaggtgacaaccgcagagagtcagaacactctgggcaacagcatgactgtccatcacgctcatccttctccgaagctcctggaccaaccctttcatggctgcctccatttcttcctcaaaggctggctcctggctcacggaacggtaccaagataacacaaaatctcgaataatcatctggatggtgcggttgatctcccgttccagctgcctttctgcctcagggcatggaggacaggtggccaacgggatgaagcgttccagatgcagtcgacctgaagccactccagcgaggctggagcccagccatcctcccagcaccactagcaatgccgacagaaggcacagcagccacacgttgaccagaaggtgtatgaccaggagccagccaagcaagacccccacagccatcagcttccggctactcaacaggttattgaggtgacagctcgatccagctggagtttcctggaacggtggcactgtttctgtcttcatggctgaacggacaaggtggcttccccagatgacagccctcaagattttacttcagagttagggaaggggggcatgaactgtgtctcagatatggggcgatctgggtgctgttcagggaaccggggctccaggccctcaaagtcctacaggcactgcaaagcgacagctgcagctccgcgtctccccatggctaccactaacagagccctccaactcgccccttccagctgaggtgtggctttggaggaaaactctgtggccttcacactgccccaggcggaaggcctcttcggggcctcggggcgggcgctgcaaggccctggggcccacggacacttacacacgcagcgggcagcggccggcgaagactgggtcacacgccgccgggaaccgcgcgcccacactcagccccgacctgaagtggactcatcgcggtcctctccgggagcctcggccctctgccgccgtaaacctgggcgactgcgctccgcagccgggcctgtgtgaaggctgaccgccggccggccgccggcgacagct

SEQ ID NO: 15315 - RNA, 2389 nt, Homo sapiens
  source 1..2389: mol_type = other RNA
gctgggattacaggcatgagccactgcgcccggccacattggttaatttggttgagagcgggctcgatgtgattttattgatgataatgtcttcaatttgccttgccctcagtacaaagcagcatgttgtaccaagggttctgggctgagggacataactagggaagactgagctgtgaatttgtcccctcagtagaggatcaccctggccaagttccagttcatcttggagccttattttacatcagatgggaaaagaccttgcaggtcattcattgtcttacatgcagagctcgcatacctgccacagggttacccagcccccagtggacagagaatttgtcccataccaaaatggctgagccacccaatccctctagacagcccctatgttggaaaattctttatgttgaatcgacatctgtttctctacaatttgcactcattggagccatacagaataaaatgtctaatgctgcttccacaaatatttgaggactgctaacacatttccttcttctacttactccacaaggcttcttttcttcaaaccaaacatgcccatctatttcaaacagggaggcagtgtggagtagtggaaagaaggccaactttggagccaggcacatctgcgttcagttcccagccccttcacatcctaacacttagcgttccgagctgccgtatctctctctgaaatctgtgagtgaaaatactcatctagccaggctactgtgaggatcagggatatgttgggtgaagatccatgctcatggtaggagcttaaaatacgagaactgttacaccttcagtttgcaattcatttagttgaccttctctgaacacattcctatttgtctctgtttcaatatgtatctgctctgtagaacagaataaaatgctttctgtgagttctaaccagcataatagagtaggattagcttatttttggtacttcccctcagtctgcagtcacagtagcctttttaagggtcctgtcttactgattcagtaagtttctcaaccaaaaccccttcgttaacatgtgctcctgttcaaccaagtttctcccattatgaagtgttttagttgatttgaatctacaatgatggctcttgaaagtggcagtcccggttgtgtcttgttgtctccataaatatcctgcacttgtcatattatgggtctcaaactggggttagaaaaatatggttcttgaatctgtggtaccatctctgctgatcccataccactgttgtgaatcagcgagataataaatgcagagctttctacatgaatttttgcacagatctgaggtcttatcatgaggcggaactgtgttagacttggaatgtgacaagaatgtgtgataagccactggctgagggagtactactgcatgagatatcctgcacagtccaggatagcatctgtccagaggaactgaaagggtgcaacttcgagcaagccagagccgactttgaatttatgtgtggctgtgtgttttctcagggctccaagtgttttataccttgggtcaaattctccccctgcggaggaagctcctttctggaagtaaatcaggcacatttagaagattcgttaactctttggctcctgggggattatggccagcattttctctcttagacttcccacagcgaattcctggttgggccaagctgatatctttgagctgacttctgtactcagggttcttccaaacaggaatatgctttctctgcctaagatctgggttccatgcccatctcaacctcaatccctccttcaaggaagtttttcctaactcctcggccagacatcaataatgtctgaagggaggatttctcccgagtgccagacttggaattcctgttgtcttcaggagctctccctggcgctccctccttcccccagggcctttaaactgtttctcctccagtctgcccacttgatccatgtgggtagacatgttccatggccttcagaataagatcttttgtggggtactcagtccataaacagaaaattgccttcatcttggatgctggtgtttctggcctgtgttgtgccagaggttctgatgataggcttataggcggtagtttcctcagtgtccgtgggtcgcccccggtcccgggttggatgccccgcggtccagcaccgaacctttcggggtgcagagttgcagagccgcggagggcccgggccgtgcgcagccgaagggaggcctgcagcgccccctctggatgcagcgggcaccggccggccgccccgctcacccgctcgcaccccacgtttgttcaccagtatttcagtttacggtcagaaaatgaacacagacacttcgtgatactctacacttttcaaaggcgtaagggatgccttttaa

SEQ ID NO: 15316 - RNA, 1254 nt, Homo sapiens
  source 1..1254: mol_type = other RNA
gctgggattacaggcatgagccactgcgcccggccacggaagtcagtcttcttagaaggaatcacggcactagagaaaatgatgatgggagcgacaccgtatagaaagacactttattacactgcccactcacaccaggccgggacaggagtcactccttagaaccccgagcggctgtccaggctgatggaggaggggaccactcacccgccacagagccagccccctcacatggcttcctccctgaggagcatctcccacactggggcttccaacgatctttgctctgcgtgtgctgaaaggacagcgtccagaatcagcctcagcctggacttctgttaccatgggaggataagcttgtcatgctcacagatgtgcactcctagtgccacgcctctaaacgtcccccagacggcattggggctctcgccggggagcttggctactgtctcgatccccggccaagcaggcctcatggccaactttctcagtgtccacagcagacaaaaatgtccacagccagagctccaaagctctgccggccctggtgccactgccacctctgcgtccggagcctgtggggctcagctctgctgctctggcccaagtctggcctggagtccctggtgccctttgcaagcacggaggcggctggacatccttcgcatcaccagcctctgggcctgcaagcgcttccggagcttttcattttccttcagagtgaggaagagttttttcttcagggaatctaagtccaaaagggcatagctgtgatcagatggctgcttgttgggggtccttctcaggcctgcagggccagtcggccggccaacagcctctgttgcttgcggcctccgtggcgagacctgttttacgtggccttcggcatttgggggcaactgaagctcttcaagtgcagtgtccatgtttctcccaggactgtcctctccggcccccgcctcagggaggaccttttctttctgagaagagctggcatttcctctctcactggcagggtctgtgttctccctcacctgcccgagcacctgggctgtgccaggcagcgtcctgggtgtggggcctgaagcagggaaggcagcccctgccctcatggagattctgtgtggggtcctgaaaggcgaacaccgtgggcacggcattgtgctttaggttcttgcggtttccaaaggcgctgaagcactctggccggaagtgctcggagcagatgaccgtgtgctgcttgggcttgaagtt

SEQ ID NO: 15317 - RNA, 1681 nt, Homo sapiens
  source 1..1681: mol_type = other RNA
gctgggattacaggcatgagccactgcgcccggccacggaagtcagtcttcttagaaggaatcacggcactagagaaaatgatgatgggagcgacaccgtatagaaagacactttattacactgcccactcacaccaggccgggacaggagtcactccttagaaccccgagcggctgtccaggctgatggaggaggggaccactcacccgccacagagccagccccctcacatggcttcctccctgaggagcatctcccacactggggcttccaacgatctttgctctgcgtgtgctgaaaggacagcgtccagaatcagcctcagcctggacttctgttaccatgggaggataagcttgtcatgctcacagatgtgcactcctagtgccacgcctctaaacgtcccccagacggcattggggctctcgccggggagcttggctactgtctcgatccccggccaagcaggcctcatggccaactttctcagtgtccacagcagacaaaaatgtccacagccagagctccaaagctctgccggccctggtgccactgccacctctgcgtccggagcctgtggggctcagctctgctgctctggcccaagtctggcctggagtccctggtgccctttgcaagcacggaggcggctggacatccttcgcatcaccagcctctgggcctgcaagcgcttccggagcttttcattttccttcagagtgaggaagagttttttcttcagggaatctaagtccaaaagggcatagctgtgatcagatggctgcttgttgggggtccttctcaggcctgcagggccagtcggccggccaacagcctctgttgcttgcggcctccgtggcgagacctgttttacgtggccttcggcatttgggggcaactgaagctcttcaagtgcagtgtccatgtttctcccaggactgtcctctccggcccccgcctcagggaggaccttttctttctgagaagagctggcatttcctctctcactggcagggtctgtgttctccctcacctgtgtggggtcctgaaaggcgaacaccgtgggcacggcattgtgctttaggttcttgcggtttccaaaggcgctgaagcactctggccggaagtgctcggagcagatgaccgtgtgctgcttgggcttgaagttgccccggccgatgttcagcacccattccttcagcagctccgggcggctgaacggaaaccggtggaaggtgagctgcttcctgcggctgctgtagcggttgcagcactgccgggccgcgcacgacttcggcatctcgagccaggcctggctgcccccaacaaagatggcggcggcggcggggcctgcggagaggggagggaccccattcgccaatgctggtcgcctttcacctccttgctttgagcacccaaccaggacgcatagccactcacaggcttggacaactggaaaccaacggccaacccctcagtgtttttagggctttgaattgtgaataggtctggactcctctgacgtcactggaggtggtactagttggccactggtggtgtcagttcagaggccagacagctcactgcccttaagtttggtcacagggaacccccaaacgtgaagaggcaaaaagggcaactgaaggggagggagattccagttcaggccttgcagaaact

SEQ ID NO: 15318 - RNA, 1193 nt, Homo sapiens
  source 1..1193: mol_type = other RNA
gctgggattacaggcatgagccactgcgcccggccagatctcttctttcttaaagtttatactactgctaactcatctccgcaaacaaacaactcgatgggcctctcttaatcctccccagtcactcaacttttcacctccaattttcttctcagtctgttcagataaatctgtttcttcctcttctttctttttcggtggagtggagagttccgtttatgttaaaacattacccaatcaacagttcaaagcatcctcttgagacagcagtagagactgcccattcgtctccttttctctcctatccaacaaacccatcgttctgaattaggtgtccctcctttgtcttctttttgatttcccattgtaacttctgcatgcctccttgatattcttgtctggtctcaactaatccttggagctctctgagcactggaatcatgctgatcattgctgtatgcacagtgcccagaaaggtgcagagataagtcttcaagagtggcccctcaggatcccatgtcagtttttcagtgaatctctcggtgtttctctctgtatgaggagtcctcctcaggcctgcttccttcaagaacacaagataactgccagcaggtaaaagcagccacgtgcttcctccttaaggtccaaaggagttcctgctcccacataaatctggagtatgacagttacaagataactcagtccaatctgtgtcccagagaacggtgattggctcaagcctgggttatctgacaaacccctgtgaaggaggggttactcagattagtttcacccaatcaggattgatctcggagccggaggtggggcccagctctccaaacagtgaactgtttcataatgggaatgaggtggggaataatgttggagagacaaatgcaagagtggtcagcaaaagtactatatccaaagacttaaaacaggattttgcttcaaaaaaatctgttatcacagtgtcttgaattcaatatgataaaatatgtagtgattatcaattatatcaatatgtaatgagtaaataacttcactggtaaacactgtatttactttttattcaaattttacaagatagaatgcaatccatcaattcaagtatagaactaaactactggccaggcgcagtggctcacgcctgtaatcccagcactttgggaggctgaggcgggtggatcacc

SEQ ID NO: 15319 - RNA, 3037 nt, Homo sapiens
  source 1..3037: mol_type = other RNA
gctgggattacaggcatgagccactgcgcccggcccacaataaaacatttttaaaaatcagaacttttggcataatctatttcgctttcccaggaaaagaaatgtagcagattttataacagagaagagaaagtaaagtcaagtcaagagtctaaggtatttccatattatcatcaaagttgccgggagaaggttgggggtcaaagctaagattccaggttggatgacctggttttgtatccaagcacagctcctcagtactacctgaccttaggttggttacttaacctttctgagccttggttccctcattggcagagtgagcataattccattcatccagcagcatttctgtatagattaaagaataaatatggtgcctggcacattggcatgaacaaacagttaaaaacaaacaaaacacatttttaaaaagatattactttttctatttagtacaaaaatgaaaatctagtgtcttcccttgttttctgagtctcgctctgtggccaggctggagtgtagtggcacaatctcggttcactgcaacctctgattctcctgcctcagcctcctgagtagctgggattacaggcgcccaccaccacgcccaattaatttttgtatttttgtagagatggggtttcaccatgttggccaggatggtctcgatctcctggcctcgtgatccacctgcctcgacctcccaacgtgctgagattgtaggcgtgagccgctgcacgcggctgtgtctgcctttgagaagcttcaagaaaaacagtgggcatgaaattatccagccctcataatactgggaaactattttcctaacaggctaattaataaagtcttacttcagccagaagctcctttcaaattgatgtaggattcctgcttttagatgaaattattggccaattatagctcagtctggtccttgggagaggtggggtctgctgctgtatttgtgacctctgatttaactgtgggcttctctctccctaaaataaaccctgggggccctgtgagtcctgcctcaccatctctggtcagaggcatcagtagggtctctccagcccccattcaaaagcatctaaccccctaaaccaggtccagatggaatccagaaagtacaaatgggggtcctccaggaaacactgctatttcagaaacaccaatggaaattccactctgacagtgacggcagctggtggtacaaaattgggcggtgtctccgcctaggcaggaaaaacaccagctccaggcagtcagccgttgccttacctggagggctgatcaaccgtcacaaatgtgtttaaaatttctaccccctccccacacccagccatgagaaaataaatgtattattgttaataaatgcaatttggaagtctaaatctttcaaagggctgagtcttgaagataataaaacacattctgggatgaaaaggcagagggctggagcccaaggctggtgtgagcagagcagtggccggctattatacttgtccttcttgggtttaatttcatctttcccatgaatcatcccatgaattcacaccttaagctcactgggccttagcttgtttattgggaagaggacttctagaggtacttctagatcagatatcctaagttccagctcatggggtcagaagtccagtgtaaggcacttgagtgctcaaatgccacctcctcagagaggccttcctggaccacccatctcctttaacgcagccttatgggtcttcatggcactcatcacaccagcagccatgcctttgcttgaaggcttactactgactgtctcccccagcggaacagaagccccacaagagcagcataggtgatgtgtctgtctagttcctagaacagaacccagtacagagtcggcattcatcaatgtgtgtggaatgaatgaatgaatgattagccaagccaagggtcaaccagaaagacagggattccaatcttacaccttcatttgctatctgggcacctctgggtaagccacataacccctccacagtattgtgtatttgcagaaaccacccccataactctggttaacatcagacagtagtggccaagtgctgctcaccatcagggacatttgtggcagtaataagcctcctggggctaataagccattggtcgatacaagtctggtttctggtacagtgggtgcctctcagaccaagatgcacatcttgctggagtctatggccactggtcaatctcagaggcacattctcactcccatatccaaccctgccactcctgatgatgaacaccggccgctgaaactgaaggaagactcctgagtgcctacacatgccaactgcctgccctgaatgaagtacccttctggctttaagagggcagtcagcgttccatttccgctcccactactcccaccccaaagagcaaccctggagggctctcctctagaagccttcccagactcacagaccacacctaaatgcaaagacacaccagtacttttaaccaagacacagaaaggcatgtctgcaacagagccataaactagacaagggctaaaaagaacagaactgctcattatggcttcaggccaacctctgcagataggcttcatcaggcctaccagagacagctgaaagcttcacaaagtacaggcctgcccagtcttcagagaccacaaccagggtacacccaaatcttcatggggaaaggaagacgtgcagaagtggaaggaacgcctgggtggctgtgaaggccagtttctgaccctccatatggaacagccccctgtgccagaacagacaggctactcccactggcagccaggcaagaggctggagaaccacatctgccatcgtcacagagctcttctatgtccccagctgcaggagagtcacactgggctctgtacaccgtcaatgctgccctctggcagggggtatggacatataaaggagcactgaccagacagagagaaagccacagatgcacacctaagtgagtgctattggacttggctgagaggcgaacgctg

SEQ ID NO: 15320 - RNA, 4157 nt, Homo sapiens
  source 1..4157: mol_type = other RNA
gctgggattacaggcatgagccactgcgcccggcccacttcttacatttccaggtcattctttctagttcccctactttaacacacctataatccactggttgtacattttcactatccctccccccgtctcaagccctcacttccctgcttacccagctgaaattccacagaccatcatcataccctgcccctcttcatgtggtcattcactctgggcaaaaccacagccctggtgaaatttatttcatctactctatgcctgcacccaaacagctttacacggttgaagaaaaacatacagccatgctcatcattggtctcatttactttaaattcattatcactaaccttgaggtccttcatcctgtctgcctataaaattgtttccaggttcatgcactttcccattcttctagcccagagctttcctctagttcctgtctcctgtatctaactgctacatgagatatttctcctttgaatagaaaactgagctcctgaccagccttcttctccaaaccaacttgctcctacaagaatcttcctcaatttctccagccccagacatggttctctttatctcacactccatgaccaaactctccccaggtcttgctgattttacctttaggatatacctagacctcactgctttataccacctctacagcaaccacctcagtccaagccagcatgctctctcaactagattactgcagtagtctcctagctgttctccctgattatgcctttgccaccacacttcagcctactcagcaaagcagccataatgtctcctactaaaattacatccctgagctataggatactctgggtttccattcttctttcactttaataaatgccattcttttattattattattattttgagacagaggctccctgtgtcacccaggctggagtacagtggctcgatctctgctcactgcaacctccacctcccgggttcaaatgattctcctgtctcagcctcctgagtagttgggattacaggcgcgcatcaccatccccggctaatttttttttgtttttagtagagacggggtttcagcatgttggtcaggctggtctcgaactcctgacctcgtgatccacccgcctcggcctcccaaagtgctgggattacaggtgtgagccactgtgccctgcctaataaatgccattcttatactataaaagactattctgtgccatcattatttcagactgttctaaattatattattattattattattattattttttgagacagagtcttgctctgtcacccaggctggagtgcagtggcgcgatctcggctcactgcgagctccgcctcccgggttcacgccattctcctgcctcagcctcccgagtagctgggactacaagcgcctgtcaccacacccggctaattttttgtatttttagtagagacagggtttcactgtgttagtcagggtggtctcaatctcctgaccccgtgatccacccgcctcggcctcccaaagtgctgggattacagatgtgagccaccgcgcccagcctgttctaaattatttttgataaatcttccgtctcacaagcaaatcaccttaaaaacagttgcatacattttcagtaatgcattccagactagaacagagataggaaattgatgactttcatgggatagaaactcatgatggcctaactgatacaactaagcttgtcaattagatctagtatttagttcaccatcatcaaactttcaaatatatatattttaaaaaggaacagataattaatgttaccaattcattttctttaggaatcccaatgtgccaaaacttgtattttaaaactaaagaaaagatgatttagacaaaatgtcataatttcatattatattctcaatgctttcaaagcccaacagtgattttaaaaagaaattaaacaacatgctttcattgaatttttaaaaatctatacaattcaagctaatgaaatattttattgtacataataaaagtggtgtttttctaaaaaaaaaaacaataaaataaaataaaaaaaaaatttccaggcccagacgtctgtgggagtacgtgaggaaaggattccactcaagtataatcagcaatactctattgaatgaaaccataactccacttcactccctatggtaaatactaacattcaccacaggcttgaaattcctgtagcatcagtagaactatttttgaaaatattacaaacatgcttatgatgcataggaggatgaaaaaatttagactgtaaccgcacaccatatgtaatcccagcttttctaatttacaaccagttaagaattacaatatccaaagaaagtattttaaaatatatatgctcactggtaagtgattttctactcaaataaataggaaaatttgcattttaatgtcacattgaatttcagtacttttcaatccaagaaaaaaaaaataaaccgagacatggtcatgagttcaggattatatatattacaatttgccttgttataatacatttgtggctttatgataaaaataactcagggacatatggaattcaagctgatttgcgtaactgtcacaagaaaaaaagcattaaatgcatttctgaaataagtattttcattaatttcagaatctcaaaacagcattagaccttgccttgtttaaaaaaaatttagttcaacactaagctagctaaataaccttcttgaaaggtttaaacacaattgatatagaaaatgctttccctctaatctcaactttacataaatggaacaggtgaggaagaaaaggtagacaatttctttagcagcatatatggctaaatccatcaaccaccttaaactagaatgtccattattgaccccattaaaaagaactggggaaatatcaaaaattactgatttcataaaccaaaagacatcaattttagggttacagttagtaaaatatttttgagacacttcaaaaacttttaaccataaactagaagaatcatctcttcattgtaagaaagaaaggcctaacagaaagacatttaaactaaactgattttcaatcctcttagaacaaacaaaatgaaaaataatggttgattagctaagctttgtgctctaatcaaactaattaattacagtgattttaaatggcaacagcccatctgactgggcagcttgacagttcagaatacttttgcaatgattttttaacgcaaagacactaaaatgatccggtcatgcaatgttcatcttatgcattctgcatctctttgccaatcttgtagctaaggatcttgttccaatcaatcttagtgcgtgtaactggcaactgtcgacgtaaggctttgaaagtagtgtccgacattgtctgataattctcactgatggcagtctggtattcattttctgcagcttctacaatctttataaattcttttgctgtttgcacttcattagacactgttagggaatcttgtatatctttatgactcactagctgaacattaccatcttcataataatgaacctgaattttcaagatgccaaccacttgagtggttgaaggagtgattgtaaacttccattctgacctccaacgaccattccaaaaattttttgcttggaactgatggctttctatgcatgcaataatggtttgctgtccatctatttttttgccatacacagtgcagactccattcgggtaatgttcttttacgtaagctctcagagcagtttctactgaagttctccatgattcaactgcattttctacttcacagggtcttggatcagttgcctccttccttaagtgatcaaatttaaaacagattctgttctttggatccaaaaactttccatttcccaagtcgccatgttctgttatcaatacctgatcttcataaccttcaatttttactggagtaaactggtccaagttatactgtgcaaatgcatgggctgctccttccctgagaagattgtcattattaagcagtaaccgaacatcattgaaaacctcattaaattctccaggaggggcatgaatgatgaattttgctgctatacgcaccttctcttcatcagacaactgctcctccagatccgccatcttccttctggcgacaaaccgcggc

SEQ ID NO: 15321 - RNA, 8509 nt, Homo sapiens
  source 1..8509: mol_type = other RNA
gctgggattacaggcatgagccactgcgcccggcccagtttaatgattttgtacactgttttagttgatactgcagaacacatattcacctttgatgggctacaaaacttccactcaccccttgtgggttctaagtcctaaaaaaaagaacactctattttcttagagaagtaattttggcaaaaggcgactgcctagctgtttcagaatgatttcagaatgatgcctgcattactcaagcaggacaagaagaggaaagcattttaaaaaggaagttgctcttaaggagaaaaaaaaattaaaacagcctttcttctaaaactcttagagaaaataaaagtaggacataggaccaaccattatgtacatgaaaggggctttttgctacccatccccattcccagcgagaaatactaagtaaactccttggtgaaacttcagctttctggttcctgcgtgtggtggggcctgcggtttgggatgctgtttctgcacttgctcactgttgaatttcaaatactctttcgtggccaggccaccactggttacctgctggtgcctctctctcttaggatctccagaggtctttgcagacacgtgggtcctcagtttcagggagctacacaggtacaggggaagcagaggctccatgaagactttggatagaaacatcttccttgacacgtcttgttccaaacagcatgaaaatggagcgctggcacacagccctcgtggcgacttctggatgtgtttcctttgctctcctctctttccctccattggaagttagggacacctctgcactactcactgacctgaggtttatactccaatagtggacccctacccgctgcgtagactccgtaagcagacccccgctctggcttcagacacatttcctgagttctgacttttccacacaataagacattctaatctgagattcataattaggtaaacctgtgtttggccctccgcggactttcctctgacatcttgggcccctggtaaaacctagtgcgaaaggggacggcaattttctccagtcttctatgtggattttcaacctgatgtagcttctgtttatgttgcagataagaggtggtttcttgtaaggtagacttccaacaaatgttggatgtctaacaaatgttggatttgtcttccaataaaagaaaggatgtcaggtttaccaacccttttcagcagaatagaggagagagatttctttgaaggagtttgtgttttgtttttcaataattactagatttatattctggctgacctatagattctgaagaaggatggattgttaaattcaacaactcccttccgcccgccatttatttaaacagatttatcatgaccattatgtaggcatttgattagctactagtttgttactaagaagtagaactggcacacgcctataatcccagctgcttgggaggctgaggcaggagaatagcttgaacccgggaggtgaaggttgcagtgagccaagatcatgccactgcactccagcctgggtgacagaatgagactctgtctaaaaaaaaaaaagtagcactcaagctcagtaaaacctggagctgagattttactgtttagattagatagatataaaaagttgttaggtttagttgttgaaacctattgttgaaaactttaaagtggctgttaaattgtgttgcttgtccacgtattaaatggctgtattttcttaggttaatgatgaatgcagacacaggactcaaagtacagctatttttctctttaatttgttaaatcaatttggagtgtatatgtggcttgttagttccttgcataggtaaggaagccaccgtctcagctttcttaaagttcagccttcctggattcacactttcgtcagttccccaattatttcccactctctcacccgaggaaagccagtcagctcagtgtgacattcaagtctctctgtgagtgatccctcacctgccttcctagcattatttcttattgttgcatgtataagtcatgcataaatcatgtgctccaggcaaactagctccttgctttctcttaatggaggcacagcacaaattcttagccagaggaccacaaactagtagaccttattcatgccgatcctttgcttggcatgcctttctctcatttctacttgataaaattctacccacttcacaagttccaacacaagtgtgacattctttatgacctttccagaggaagaaggccttcttcatatttgaccccccacagcacattacaagtccgtcatctcacctgacacattcactattgttctttatttatatatcccatttcccctatttgattttcctttttaagagacagggtattcttctgttacccaggctggagtacagtggtgtgatcatagctcactgcagccttgaactcctgggctcaagtgatcctcctccctcagtctctcaactatctgggatcataggcacatgccaccacaccaagctctatttcctctacttcttaagagctggatttttatctgacttacgatatcaatatctgccatagtacataataggcactccacaagtaattgttgaataaatatttcattttcctccaattcattcattctgtcaatcatcaggtatttcttgaatacacactatatgccaggcacatgtagctagcaaaatctaggtttgaagcttacctgtggattttaatgatctatgctatttcaaacctctacctgcatggggaaagatttgttcttatcatgcagaagtacttcttcttgtcattaccactaattctattatttttcatggtgtcactcattggcaaatttagtaaagcatgtcagggttctgcatttatgtactaaatatacgtctagttttgtcttatcctttctgtttctatttttgtttgctctgagttcctcacttaatttttgttttgtattatatatattttagtagctgcctcaaatccttttgaaatgaagcagagtaccaataaataagtagaataaaatctgaagaaaatcaagtaattggctccaaaccacaaatccacacaatgaaatctcactcggagagcttttgctattcagaattcaataaaatgtaggtcttccttggactcccttcaaggggcaaagtttctaagataattataaggtgatcttacttttaatgtgatcccacacatacatcgtttagaaacctgttaagaaaatagtaatattgtcattgtagtgattgatggtatttgaaaactgcattgtaaaatctgggactgttcacagaagcaggtaaacctgaggacaaacatgtctatgtacctgaaaatactttttctatcttagtgattttttttttaaaactaaggttgctagggaggtgatttatcaactttagaaaaataaagggagctaagcttaaaatatactaatatactatgtgggaaaaatggctcctgaaatgagagtgcttaatagaatctgcatgaagtcaacagcaatggtgttaaccaaagcatacattttccattcccatcctatagaaattgcattcatctgccaccaggctattgttactttaatacttaaacctcactagtaaaaggaagctctttcacccacgttaagattttgccattttgcactcctatttctctattctcatgcttaatgaatacaacccctcctcatctatctagatatgtatcaagcttaacagattctatttacaccaggcagatttgttgagtcctatagccaattcaaaactttgttttcaaaagatgactgataattagtttataattaattcctaatgctgtatttcacagagtaggcactgtatctttatggttaactctagggaagagaaaacatagcattgtcaagcatgatattaaaatgacaaaatgacctcaggaaaccagagttctaaacaatgactacagaagaataaaaaatatctagaaaattgcagttattttagtttaatggtatacattggctatgattacgatatgtaatttatttaaagcatattttttaaaaactagtttcaattcatctttatatgtatgttaaaacccagtgcatcagcctggagacttgtcaagtttgttgttttatctgcatttaccaggctccagtgctgctcatccatggactgtagcccccaagggcaagtgccatgcttctattcattcctgtcacttagcattgggtctattctcaaccagtgttagttgaatgaaaaaatggacttttacctccttgccataatcctaaagcatgccaagatggcatgagcctcagcctttcagaaagaacagacttgagtgctagcgaatatgttctggaaaacgtttggcatactgatacatccaggagagaaaggacaaggaatttcttcttttgtccctctttcaggaaatcctcacagagattttattaatagcttgattaattttaatagcttggttaattctatgatagcttgattcaaattgtgccttcacatacatttgtacgtatctcagtgcagccacaggaattcttgtaacccaagagtagaatttatattgtagcccatgtgtgtttttttcctttgcaaattctctcatctattctatttctgagaaaattcttttaatagccccttttatggcccaaatttacatcttaccaggtagatatttctctgggcttcagtgaaactactctgggaaataacaggaaaaaaaaatacacctctgaaagtgagctagccccaaggaataaggttcagaagtgaaatgtgatctcatggaatgcaactacctaagtcgctatacttcagcctattttgttttcagagtagcacacaccaatcaagtggttgcctatctcaaaaactttagaatttataattttagaaatatgaaagagaatttgcaatgtgatctcagtggctggctcacttctccttgtaaaaatttttatctgattataaaacaaacaacctactttttcaaggcatatcagtgccatgaaatcatgctccacctttgcccgctttcatcatatcaccaggagctgcagtctgatataagagaggccatgacagagagttaatttctgccaatgcccttctggcttttaccgcaagatatggttatttaattttcttctgggcatttacatagagctttgatggtgcttcttaccatatcactgggtctgcctgactgctttatggtgaatctgaaaccattgggaaaatggtccagagtccctgaactttgctggatcctaaaattatagtttggaagctgtgagaatgttggtgaataaaaagaagcatgtgtcttttccatgaattaattttgggtgagattgcaggataaaatgatgcttgctcaggaagtgccaatgcccatctacccaccctgacctcggggagcagcactcagcctgacatgccaagaacagagctttgtccccatgtctcaggtgactgaaattctgccttctgcccagagcccctgcttgggcttcaaccagcaaagcaaaggcctaggaaacatttggtaccatcagctctggtggttgcacctaagatggaatttcatatagcctcttgtttatttatttattttatttaacaaggcgaccagttaggggacccaggttaagcccttcaacagaactatcctgaagagcaaaagtagcaaatgacaggctatgactagggattgaatttggggaaggctggatttgtgaaatgagagccaaaaaagttttcaccttctagcccacaggttaagttactgaaaatcagtcatcaccatttctacccacttgtgtgtttctcctactctggagagtaatctaactcatcatttgcaatcagggcctctgagttctgtttgtgtttgcttttgctcttcgctttgctacttgtccggccgtttgccttcgcatctgacatctgttggtaatagaagcctttgtcttcagtgggcccgccccagtcctcctggctctcgccctctgtggcgtaggagaaaccctcctccactgagaaggggtcatccacgtcgtagcgttggtacgtgctttggtgcagggcctcttctcgagcgctgatttccagggtgctgttccagatgccatatccaaaataaatgagcagacccacaaagcaccagaccgcaaaccggatccatgtgatggtggagagctttagcatgagatagatgttcaccagcatggcaaaggcaggcacaaaggggaggcaaggggccatgtagggcagcttcttggggttctctggctgctgcaggatcacaaacaccagggtgctgatcagcagcaccatcagaacaaccagaaggatggcccaccagctctgctctgagatgtagtcagaaccaaagatgatgaaggagcagaagatgaacatgaggatgaagagcaggagcacgcagatggtcaccgtgtgccccgtcgctgctgtgggccggtccattttgcctggaaggcccagccggattctcatggtgtaataatgaggcccaatcagcttctttaacttgatgagataaatattttcggattcatcagcttctatgcctgtggtcatgtccacggtgccgtaattggggtggttgacgttgtaggttgacttgtctgatttccctatgagcatctcattgtctcccaaggatggtaagttcttggccccacatgtgttggtggctgggccagaaaactcatccccctcactcacaggagaacaagcttccttctcacagtcagccagaatgccctccttcttcttggtgtgctcctcagacaagaacttgacaaaaccatcaatgtcactctcaggttggtatcgaaggagcaagacacagacagagaccaaggtgtaggccaggagcgtgccgatagacatcatctctatcaggtctctcaagctgaccaacagtgcgaggagcgctgccaggaaccccgacacgatgcaggccaccactggtgtctctgtgtaggagctgacgtgagccaggaacctgaaaaggagcccgtcaccagccatggcataaatgaccctcggcatcgggaagagggaccccagcaagctgactgtcagtcctgcaaccgacccaatggccactacgaatttggcagcatagaacccatgagccacaaacatctccatgagtggggattccgtgtcaatggtataatatggcaccatcagagttaagatcacgctcacagacacatatgctgtcaggcagatgaccagggaggcagtgatagcataagggatggacgtgttgggattcttggcttcctctccagtggtggcgatgatgtcaaagccaatgaaagcgtagaagcatgttgctgctccttgcagcacccctgaccagccgtggggcaagaactggccctccgcccagtatttcccattgatgaagaagaggcctgcgatcatgatgaacacccatactgccaggttcagcacattgagaacattgttgaagcctatggaattcttcacccccagagcaacaatgatggtcacgatgaccgcgatcaacagagccagaaggtctgggtatgattcttcacctttccccaggccattgagggttcccacgctgtccgccatccagcggctgatggtgtggttggctagtgagtcaaacatgctgctcagagcactggctccggccgcagtgccaatcaggtactccaggatcaggttccagccaatgaaaaatgccacaaattccccaacagtgacatagctgtaggtgtaggcagatcctgtggtcttggggactcgaactccaaactctgcatagcagacgcctgataatatggatgcgacggctgcaatgatgaaggacacaatgacaccaggtcctgccatttccttggccaccaggccagagaccacatacatgccagtgcccacacagctgccaacgccaagagagatgaggtccactgtggtgagtacctgggctagcttagttccatgtgccgtggtggtcccagttccctctagcatggactccactggtttggtgcgtaggatcctggagtgcattgcataccaggcagctccccactgcacccgccgggggtccagcgaggtgaagaagccactcatcttgagcgataggggatgcagtgaaggtcagctgatggaagggggctacaaagccttagtggatggttctggaactcatctagtgaacagggatctcccttttaggaaaggcccagagggacccagtgcagccttctcctgggcatgaatgtcggggtcggggctggaggcgacgagctggctgccaaggctggtggctggcagtccgcacttactgcgcggagctgtctctctagctgggatgggaagtggtggtggcggcaaaggaaggcaggaggcagccgctgctgctgaacagctcctcaattattcagatt

SEQ ID NO: 15322 - RNA, 1216 nt, Homo sapiens
  source 1..1216: mol_type = other RNA
gctgggattacaggcatgagccactgcgcccggccctgctgatgttgaacaggttttgccactgcctggtaccatactcgtgatgagggtggctgttttaggggagccctgaatcagcagaggggaccagtgcctgcgcacagaagtcttagggcacgtcccagccctttcttttccctcaacatctcctgaggagcctgtagtcactctgacactgtcacagtgcctctggagcccctcctttccctaagtcccatccacaactccttgggacaaatggttttgcatcattctcacctggcccaggtctccttcttgtccatagggctgttatgacagcctttgacggacacctctctgagaccaggtgccatgcttgaccttttcctgagcagctgatttgcttcctgtcaatggaaagcaacgcagctggtctggtatgtctcattcttgataaatctcttcgttcttttgaacccgctggctccagggatcatacttctttctgaaaacctgagttgttcccattgaacttgccagcggccttgtcaggaggtttctctgtttcaatttttagttctcggctccgtgagggatgagactggaacacgatgctgcagccctgctctctcctcagtgaaggctgaaggtgtgtgacatggaaggtgagaaggtggcacagacggggtcgctccatgagaggaggagtgcaaggagagaggagaggcggccagagggctcagacctccaggaccctcaggggagggggcacgaagatgagccaggaaaaaccgtgagaaggaacagcgcaaggccggctggggccagagccaaagagagggtcatcggccgcagaggtgggtgacggtcctgagcgctcactgctgactgttaggcgccactgagggtattgcactctcaccattcaatgccatgaaagggagggaggaggcagcgctgaccagctagggaaagatatttactaaacaggaatatccagcttaatatggtgatgaattgctcagtttattccacctcttgttgatttcttcatgatattggcttagggcagagatggcacatacatggcaacatccttgactcccttccatctccctagaaaacaacatggcagacatcacaatgttaccgggggtccttgctcccagagctcccaacatggtggcgggttgcttccaagatggcagcaagcctc

SEQ ID NO: 15323 - RNA, 1303 nt, Homo sapiens
  source 1..1303: mol_type = other RNA
gctgggattacaggcatgagccactgcgcccggccctgctgatgttgaacaggttttgccactgcctggtaccatactcgtgatgagggtggctgttttaggggagccctgaatcagcagaggggaccagtgcctgcgcacagaagtcttagggcacgtcccagccctttcttttccctcaacatctcctgaggagcctgtagtcactctgacactgtcacagtgcctctggagcccctcctttccctaagtcccatccacaactccttgggacaaatggttttgcatcattctcacctggcccaggtctccttcttgtccatagggctgttatgacagcctttgacggacacctctctgagaccaggtgccatgcttgaccttttcctgagcagctgatttgcttcctgtcaatggaaagcaacgcagctggtctggtatgtctcattcttgataaatctcttcgttcttttgaacccgctggctccagggatcatacttctttctgaaaacctgagttgttcccattgaacttgccagcggccttgtcaggaggtttctctgtttcaatttttagttctcggctccgtgagggatgagactggaacacgatgctgcagccctgctctctcctcagtgaaggctgaaggtgtgtgacatggaaggtgagaaggtggcacagacggggtcgctccatgagaggaggagtgcaaggagagaggagaggcggccagagggctcagacctccaggaccctcaggggagggggcacgaagatgagccaggaaaaaccgtgagaaggaacagcgcaaggccggctggggccagagccaaagagagggtcatcggccgcagaggtgggtgacggtcctgagcgctcactgctgactgttaggcgccactgagggtattgcactctcaccattcaatgccatgaaagggagggaggaggcagcgctgacctctctgaaaacatcgcctctggccattgatttccaggaatctgcttagtgcctgcacctcctccccctcacaggatgcaaggataccagctagggaaagatatttactaaacaggaatatccagcttaatatggtgatgaattgctcagtttattccacctcttgttgatttcttcatgatattggcttagggcagagatggcacatacatggcaacatccttgactcccttccatctccctagaaaacaacatggcagacatcacaatgttaccgggggtccttgctcccagagctcccaacatggtggcgggttgcttccaagatggcagcaagcctc

SEQ ID NO: 15324 - RNA, 1892 nt, Homo sapiens
  source 1..1892: mol_type = other RNA
gctgggattacaggcatgagccactgcgcccggccctgctgatgttgaacaggttttgccactgcctggtaccatactcgtgatgagggtggctgttttaggggagccctgaatcagcagaggggaccagtgcctgcgcacagaagtcttagggcacgtcccagccctttcttttccctcaacatctcctgaggagcctgtagtcactctgacactgtcacagtgcctctggagcccctcctttccctaagtcccatccacaactccttgggacaaatggttttgcatcattctcacctggcccaggtctccttcttgtccatagggctgttatgacagcctttgacggacacctctctgagaccaggtgccatgcttgaccttttcctgagcagctgatttgcttcctgtcaatggaaagcaacgcagctggtctggtatgtctcattcttgataaatctcttcgttcttttgaacccgctggctccagggatcatacttctttctgaaaacctgagttgttcccattgaacttgccagcggccttgtcaggaggtttctctgtttcaatttttagttctcggctccgtgagggatgagactggaacacgatgctgcagccctgctctctcctcagtgaaggctgaaggtgtgtgacatggaaggtgagaaggtggcacagacggggtcgctccatgagaggaggagtgcaaggagagaggagaggcggccagagggctcagacctccaggaccctcaggggagggggcacgaagatgagccaggaaaaaccgtgagaaggaacagcgcaaggccggctggggccagagccaaagagagggtcatcggccgcagaggtgggtgacggtcctgagcgctcactgctgactgttaggcgccactgagggtattgcactctcaccattcaatgccatgaaagggagggaggaggcagcgctgacctgcagagggcaggagggcagaaagaactggtttgggctggttgtttttgtttttgccatggaggaacatgttggtccacagaggggaagcctcgggaagaaaggaaaacactgaacatgcaaaaggtgaaggaaataattgaccgagccaagtcccccttgaaggaggaggatgcgaaggtgggaagtcattgtgttaattgaagcagagggtgataccccagggtgcacagtctgatcaagtctgataaaggtggacagaagctcccagctcagcctaaaggtggcatctcctcaactcccatcccccagtctgaatcttgggatcttagcagtgcatgggcctggagaccaaagcaatgttaggagaaggatgaaggcctctctgaaaacatcgcctctggccattgatttccaggaatctgcttagtgcctgcacctcctccccctcacaggatgcaaggataccagctagggaaagatatttactaaacaggaatatccagcttaatatggtgatgaattgctcagtttattccacctcttgttgatttcttcatgatattggcttagggcagagatggcacatacatggcaacatccttgactcccttccatctcccatagggcacctctttggcccaattcagggctccgccgtgtggctcggggtgggccctgatgagcaggggaggggatgtagagggaggcccaggttgacttgtcccctggaacagtgctgtccaatcaggggggatgctgactgtcccgttaggagcggggcggggcgagagagggtggagaactgcctggcaggcgagctgtcctggcgtgaaaaggctgggctaaaaggtcccctccctgctctgagtctacattctgagtctgggcttccttgtatatttgagaaacgttaattccccgccctca

SEQ ID NO: 15325 - RNA, 1684 nt, Homo sapiens
  source 1..1684: mol_type = other RNA
gctgggattacaggcatgagccactgcgcccggccctgctgatgttgaacaggttttgccactgcctggtaccatactcgtgatgagggtggctgttttaggggagccctgaatcagcagaggggaccagtgcctgcgcacagaagtcttagggcacgtcccagccctttcttttccctcaacatctcctgaggagcctgtagtcactctgacactgtcacagtgcctctggagcccctcctttccctaagtcccatccacaactccttgggacaaatggttttgcatcattctcacctggcccaggtctccttcttgtccatagggctgttatgacagcctttgacggacacctctctgagaccaggtgccatgcttgaccttttcctgagcagctgatttgcttcctgtcaatggaaagcaacgcagctggtctggtatgtctcattcttgataaatctcttcgttcttttgaacccgctggctccagggatcatacttctttctgaaaacctgagttgttcccattgaacttgccagcggccttgtcaggaggtttctctgtttcaatttttagttctcggctccgtgagggatgagactggaacacgatgctgcagccctgctctctcctcagtgaaggctgaaggtgtgtgacatggaaggtgagaaggtggcacagacggggtcgctccatgagaggaggagtgcaaggagagaggagaggcggccagagggctcagacctccaggaccctcaggggagggggcacgaagatgagccaggaaaaaccgtgagaaggaacagcgcaaggccggctggggccagagccaaagagagggtcatcggccgcagaggtgggtgacggtcctgagcgctcactgctgactgttaggcgccactgagggtattgcactctcaccattcaatgccatgaaagggagggaggaggcagcgctgacctgcagagggcaggagggcagaaagaactggtttgggctggttgtttttgtttttgccatggaggaacatgttggtccacagaggggaagcctcgggaagaaaggaaaacactgaacatgcaaaaggtgaaggaaataattgaccgagccaagtcccccttgaaggaggaggatgcgaaggtgggaagtcattgtgttaattgaagcagagggtgataccccagggtgcacagtctgatcaagtctgataaaggtggacagaagctcccagctcagcctaaaggtggcatctcctcaactcccatcccccagtctgaatcttgggatcttagcagtgcatgggcctggagaccaaagcaatgttaggagaaggatgaaggcctctctgaaaacatcgcctctggccattgatttccaggaatctgcttagtgcctgcacctcctccccctcacaggatgcaaggataccagctagggaaagatatttactaaacaggaatatccagcttaatatggtgatgaattgctcagtttattccacctcttgttgatttcttcatgatattggcttagggcagagatggcacatacatggcaacatccttgactcccttccatctccctagaaaacaacatggcagacatcacaatgttaccgggggtccttgctcccagagctcccaacatggtggcgggttgcttccaagatggcagcaagcctc

SEQ ID NO: 15326 - RNA, 3234 nt, Homo sapiens
  source 1..3234: mol_type = other RNA
gctgggattacaggcatgagccactgcgcccggccggatgagttgtcttctagaatttcttccagctcaatcactccacgattttgggaatctgagaatggtgagattaactgggaggcaagggagaaggtgggacagaaattggtttatagcatcatttaaatagccaaacagaaggatctagaagccagtttcagttggggcagctaacttgctgtcaatttgtctaagccggaaagggagaatctgcagcattagtctgtggcatgtgagaggcccattaataaaagagccacatgtgctcaggggaaagcgagttacatggaaggacaaggacggttgtaggcttgcaaaggagcattcattaccatgcagggcgaatcaaatgaagaaggagctgagggcaaaggggaagagcagggaagcagagaagagagagtagaagatgatggatggagggactcgggagtgtggtggctcagcccacctcatcctagctcagcaagactgcagaggtgtgcactgttccccatggtgagaattgggtgtcctttgttgcttagtcttcgggttccaggaggctctgggaccaagggacagacaggaagggagttggagcaggggaggcaggagactcgacggaggccgagggcagtggcctgatccagtatctctgtggagagtgggaaggtgttgaggtctatggtacctgccagatggtagtggctgaataaaagtgggaataaagcaaagaagcaaggcaaggaggagaagcagcagcaagagagggagggagagagagagggaggaagaaagcatacaccagccaggtagttttgtgatgcgggtgaacttggactggaacagacaaactttgttgactgttttgctctgtaattgccttttaaagagattatccagagctggctcacccagttcccctcataggcctcctggcccaacatgtagcaaaactgggtaggaaataagcccatccaccctgcctgtagccccctgtccttaccactccctggagccttacttagttcagtcaacaccggcttcctgagcacctgctaacatctgtctggacctgagggggcacagcccctgccctcaggaatgctgtcttctgacgctggcagtttgcagagcacttttacagacttgtgaggcagggactgctgcttctcttttacaggtaacagaaattgttgctcacttggagggattcacatgcctgggatcactcagcacatagtgaggggctgggatctggactctggacttggtgttcatgcttttaagctctttcctcgacacctcactgtctcacactgcttacactctgcctggagagcttgaaaaaccccgagacagcatccctccatccaaccgtggaggggccggtgtcccagggctggctaggagggaggcaggctgtaagcagttggtcccctggaatggtggtctcacaagggtgctctcacaagggtctcatgtgggaccctcacaaggatgccatcagttgaaagaggaggctcggaaggggcaatgttgagtcgccagtgatggaatgtcgtgtttcagtgaaggaacttgccttgtaatgggactctgtgtggacttctagccctgtaacaccactcctcccaggaggcctccacctgccttcctggaccccctcagggccttggcacagtactgagtgtatagtcaattgcacttgctagggttttgtttgtttgtttgtttgtttgttttttgccagggaccccgcatacattaacatagtgtggtattatctcctccttagatggcacgttcctcaaggacaggtgtcttctgtctttccactcctaccacctccaccaagatacccagctttcccctccccacaggctgcaaacattgtatccacttattgggtagtgggcaaatttcagccagaagttaattcaagtcaagcaaatgtcttaggggccagccacacgacaggccccatgacagatgctgtgcagaatatagagattaaggtcctgtgtgttccctgccctgagaagcttgcattttaatagggaagatgaaaatgtgggcacacaactatgctgacctcttccctgactttcaggccccgcatggcaggacccctgccatgtgagtgatggattgcttcctccagccccgcccctcctctgccctcctctccttctaggagtggtccaactctccactttctagtctttgttcctgcagttccacgctctggaatgcctttccctcttctcagcgactccccatccttcagtgctcagttccaatgcagcatcctccatgaaagactttcttgattgcccaaccagatgtttccctctttggaaccctccccaggaagacctttgtggacctaccacactctgtctcatgttcctcttgtttgtgccctgtctcctcatacctcccttccccatcctgctgtaatcacaggaataggctcctactcatctttgggctttgaacttaccatgtgcttcatacctactcatcaagttgtacagtacaaagtggactaatattaggcacatttaggaagaaacaatatcgtggggtcttgtaggaggaagtgaccttcaactgagccttatagaatgggcagataggggggcagtggccaggttcctttctcttcttgacataagcagccgtgccctcttcttcaggattcctggtagcagtggcagttgcttgtttccccaagttcacgtagctcatcagcagagaagccgggttaaactcctgtccaactttgcgttgctggttctggttgtgcaacacccaaggatgaagtccagctcgaactctgcattcccagggtgcagtggcagggccacatcagcccagaggggtgcttttttcttatctgcattaagatgctgtttgtaggctagcagcggccctgtccaaatccataccttctcctccttcactgcaacccctggggcctctaaacagtggaaaggcagagcaagtgagagagacagaaagtatagagggagccaaggagagacattatttgaagcaaaatcaagcctgcacatgtgggcatgtggaagcggcttacaaaacagctgttcctacaggaggtttggggggcaggtgtcagcagggtggagcaaagggatttggccggaggcagagccacagattgtcagtgatgaaagagctatgtctcct

SEQ ID NO: 15327 - RNA, 5063 nt, Homo sapiens
  source 1..5063: mol_type = other RNA
gctgggattacaggcatgagccactgcgcccggccgggtcttgctcttagttttactgaggtgcagaatttactcgccccagagctgccctcccttgggacttcttgccatgtgaaataatacatcccaccattgttaaaagggctgatttttgctattggtagctaaacgcttctaagctgctggatcctgaatccagactattcttaattattgggaagcaatactgttctcttttggaaggtggacattttgcaagaccaacgtgactaaatggtcaaattctgttttctacggtagagacacagaatttgaccattattagatcattattgcgaagattattattgtgaagcaggacagtcaagagtgttcttatgaggcagggcagcatctacacgataggtatgtagttcatgtatgtggtgtctacatatgctttggtaaaatgaagctctgttgatgagacagccacatattacatttcatcattctcagggatcccacagaggctgatgttgtacagctttcaggatcactcgaaccctaggcagcggtctgaggagcttccagccacctcttagtgagagcctcaggtgtgaggaccaagcgttaggatccgccctttttttttttttttgagacagggtcttgctctgtcaccccggctggagtggagtcgtccgatcacagctcactgcaacctcgacttcctgggctcaaatgatcctcccacctcagcctcctgagtagctgggagcacagatgtgtgccaccacactctgggctaatttttctacttttttgtagagatggagtctcagtatattgcccaggctggcctttttttcttttttaaaatactgtcatcctgacttgttgaaacaaacccttttcctatttccatattaatttgtagggttgataagtgcaatgttcaatcacaattcctctggttttgtttttgggcagtgacttgcatctcccctccctcattttcattcattgaaaagttctcaagtggctgcagctaaaatcagacacttaaaattaatgcaagattaagattccaggtgatggcttcttcatgagtccatttaaaagtcttcgttgcaataaaaaaaaaacaccacaaaacaaaaaacagtgaaatccaataggatggtaagctaataggtcacggagtggcgggggggtgtctttttatcccccgggttgggcctcaagcaataatttttgtgggagacaggacaggtataggcatggaaaaccaatgtgaaaacctgtggttcatattccccgtggttgtgctctgggcaaatgtttgaggaatgtcatttgtttctgttgttgttctcaactgatttaggagaaaaaaggcactgatccaggagcacacattttctaccagctctgaatagtttaaattccaaataaaaactcacatccagtgtgtttattacttaattttaggtcatgtttaattgaaaacactccatcagccttttgaaagtaaattttgagatccagccagtggggctgatgatttccagacagcctggacagctgagattcggagctcagctcacacgaagaggcagacgatcagctgtgttcgtgagcagtgcaggtgtgcagctgtgagacggtcagctgtgctcgtgagcggtgcaggtgtgcagctgtgagacggtcagctgtgtttgtgagcggtgcaggtgtgcagctgtgaggacattccagggtcatcattaccagctgtgaccttgtgcccctgactccccgtcttgggttccttttctttaaatatgactcatcaaatgaaaacctctcagtgttgttgtgaggattaagccaaacagtgcaaacaaaaggcttagcacagtacagcggtttacagtcaatgctttcaatggcgctagctgtgaacatttggtaactgtaaccagttaactttcagggctagatatgacaacacatcctgcaaattcctccattttaatctaatcaaaatatataatgtgcaaaatacaaaataaaagaggaacacagtgtctgcttgggaaggcttccatttacaaacagcatgttgaaaaagttcacttttgtttggaggactctatgttcccatagcaacagtgctctaagtgtgtgtgtgtggggcttaaattccaaggactcacaagggcaaattaactcttagttacgtgaaatattgtgttagtcctgatagggttaaacaatgactgtacttgtagtgaaacaaagaaaaaattgatatgaaaataagattgaaatattttaaaatcctgtggctcaaaggaaagcaggatgaactaggggccaaatgaagaagctgtggggccttggggtttgagacagggcacttaattaaatgtaacgctgttttccttggtgcgagggcccccatactcatctgtattgttcagccctcaagagaatcttcactggctggtaaacgaacaagaatagctggagaaggaatacttcatatagtataaaaaagacccttggacaggcatggtggctccagcctgtaatcccagcactttgggaggctgagacaggactgcttgagcctaggagttctagaccagcctgggcaacacagcaagacccaggtgcggtggcacgaacctgtaatattagctacttgggaggctgaggcaggaggactgcctgagcccaggagcttcaggctccaagtgagctatgactgtgccactgcactccagcctgggcaacagagcgagacctcgaaaactagcaggtgagcaggttaaagctgagttctctgctctactttcagagtctttaatatgctaatttcttcatgaggttcacagaatgtcgtctaaacccaagtgaccataaccccttccttcctgcagcatctccaggggcaagagttctgggaacacacctgagacaagtctcctgcaatgccagtcttggcaagccctcctcccgctcctcagcttccccttccagcaggcaacctcccccaacaccccctctcctgctttgccttgggctacttgtacttaatccgtccagaggttttagttgatactctaatgtgatttctgcatttccatctgaaaaccaaacagatttttgacacaaaggaagcttcatagcaggatttcaggcacctttattcatggcagatatttttggtcagggcagcctgcctttgaaatcgttccattacttgaggaggtcgactcctgcctaagtcacaactctcctacaaccgcaaccggccatatcatttccatttgccacttccgaggcttgagaacatcaccagggacgcaggtttcggatggtctggtcaatgctgcagtgtgtgtggggcattcgggggctccagcctgcatcacaacctactggcctgatcaaaggaggttctgtagttgggtaaccagagtggtgaattcattttatcacagaaggatctcactcctttatgttccccatgtaatttgtatacagcacaaattatttcttactttgatagatttgcaatataaacaccaagactggtgagatgagaaacttaaaaaaatcatgtttttcaaattttcaagtttttgtgtaaaagcactttgtggtgacaatcatatggatcaccttccaggtcatcagtattggcctctaggtttagcactcctggcactgcatttttgagtggccagagataaaggtattatccctgtcttctataatcaatgataacattgacactctgcaagaatttagataagaaacagtttaagtaaaatagtgttttttaaaaacttgagtctactacaagtcgttgatcatattctagccaagcaactggcatggacttaatatggtctcttttccttctctctttcttttcaagtcactagctcaaaggaaagactgattgagttttaaaatcctgccagattttttatggtaaccattgtagatgaaccacgtaggtagggtcctactgaagtattagaatctcatgcaaaactctaacaaacgcctcattacagaaggctattctgttattttctgtactgtaaaagttctgacacaagacagtggcagtggttacttttcatcgactttagcatgtgatctcagggactcagacatacgtctaagttctattctgagttttggcaacagagcagtgacagatatttctgaatgaacaatttttaggtgttttcagccatttgaaaagtattgccaacacactatttggtgttagctcaacagtcacgttgtgccaagaattaaagaactctaaagtctacaaacatcttacttcaccaagactaactataattgaagggtttactatttgtttaataaaaaatcacacatcaacttttatccaaacagcaactactacaaaaggaatgacaagaaaaaaaatgacttcacagaaatacactaaaaaatctgacaatgttatgcaagaaccgccaaagttttagtgtttaataatgaatagcacaactgaccaaggtccaagatgtgaagataccatgttcaagaaactggggggaaatcactctacaaactaactatatactaggtgataagaatgcatactttataatataaaacctgtctacacatagtagttagctgcaaaaagccattcgatcttctcttggcttggaaaaatgccagattccagtataaattattagcaaccttcaactcttttgcgtggcaggtatcttgttttcactttccagttcttccaccccagcctgtgtcatgaggtccgcgatattcttttccagatcatcaatgcgactactcatatcatcaattctcccaatgatctggtcagacatggtctgaaatttatcttgcatctgctgcaggagtgtctgcaccaccgaggtgaggtcctgcacggtcttggggtcagtctcggccatctccccgatgcccagcttggcggtgatgtctcagaccgtaacctacacttccgtttgtccgctcagtcgccccgggccgctgcttctcgcgacgagact

SEQ ID NO: 15328 - RNA, 450 nt, Homo sapiens
  source 1..450: mol_type = other RNA
gctgggattacaggcatgagccactgcgcccggcctaacaaagttcttcatattgaaggaaaatgataccagaatgaaactcagatctacacaaaagaatgaggagcatggaagataataaacgcgtaggtaactataaaagattctctttttcattgttaaaaattattcataaaataattgatctttaaagaaaaactatgtattgtggtgcttataacaatgaagacatgaaaattgtgataattgcaacgcaaaggaaggaaggggaaaatgagtgtgtattgttttaaggttcttatatcacacatgaagtcatatactatgatttaactgtattaagttgaaggtgcatattgtaagccctagagctaccactaaaaaaaaagggaacaaaatcatatagactgtaagtcaacaaaggagttttccttgtgactcttattttct

SEQ ID NO: 15329 - RNA, 4189 nt, Homo sapiens
  source 1..4189: mol_type = other RNA
gctgggattacaggcatgagccactgcgcccggcctaagcttctaatttcaagatgtcatcagacagcagggggacagtggagtcaaacctgccaactctaccccctcccgcacactccccaccaacgcactctcagctgcagttgcctagggcaaaggctctgcaggtgcagactcctagagagccctggacaattcagaaagagcccctgaggggagaagcctagtcctgtagtcagaggctttctgaattcccagagctgcacggctcagccaaagaccagaaaagcctctgaccacagccagaaggccctgccttgtttgctaaggccgccccagccatggggctgaggaagaggagagggcatacctgagtctgggcgcccattcccagaggccacgcagaagccgaaagtgccccctggggagcgctgcagctgcagctggctggtgccgtctgggaacacctccaccaggcggcccacggtgcgagccaggctgggagcacccacgtcctccacactgagggcacgccgtggtgaagtcttggccggcctgccagctgcactgtggtcccctggccctgctaccaggtagaggctggaccggttccccttgctgctcagcagagaatggaggttctgaaaagaggcagctttccgacgctggtgagagggtgacaccgggtgcagggattgtaacgatggggccctggactgtgacgtcaggccaggcggggcgggctgcaactgctccacactgtagctgcgggacttgcccagcttgggccgggaactctggcccagggctgagaagagctttttcagccccagggtggaggctatgctgctgctccttttcttgttctggtccaaaggggcagccgagggggagccgggtcctgtgccagctcctgctgatgctcttgacagcacatgtcctccagatcctgaccctgtcctctgcaggcttccctctgattccttgctggactctgactcctctgaggacagggagagggtgatgcccgtggagttgatggtggcaacatctgctgagccaagaaagccctggggtcctccatctctgctgttctccaggggcggctccggttcccggctgcaggggcccctctccaccctaccctcgtggacggctcccccgtagggctcctgcagcccccgaggtgcgctgttgttgcagttgttggtggacagggccagcagtgggtgcctgacctgagggcggctgggctgggtctgtgatgggggcagctcacaggtcctgagaaccgcgcttcttgaaggaggccgagggatacccacaggctctgtctggtcacccagcctgagcagtccagccagggctgccttcctgtgagacactggcgaggtggttttcctcgaagggggaggggttggcgcccagccttcaggacacaaggaagctgttggctgccaggcttggtgtggggcagaaggctctgcatggctctgttgcagggaggaaggagagacaatttccagggactcgtggctttctgtaacctgggcctggcctcctggccccgatgattcaggcgtcatgggggcggtggtggcataggctgtcctgcatggagtccgggaatccaaagggtgaggctggtgacttcccagccctggtccaggctgccactggggtcccagggacacccgcttcaactccaggtcaggaggcttggcatcttctctcaaaaatagagttccttcaggcgtgtgtcctctgccctctttcacctcattttccacctccacatcatcagccctaggcaggtgttgctgggcctgaaggccccaagggagctccgcctcagccttcttggaccacctgtggcctcgaggcctggagccccgcagtcgcagtcgcgggctgctgccttgggtccgcccacacgcccagccagcctgagaggtccccgcctcctcactgtcggtcctgcagttgtcagagttgtctgtgctgtccagggcagagtccacctccgcagggcacacggtgtctccgatgtgtgtttcccggatccattccatgtggagccggggctctgcaggaaggagccggagtggggagctcaggccacccagcaccctctccatcccacaggcagcctggagctcctggagggtcctggggacggggggcgccttcccctgggcggggcgcgggtcgtcgatgcagctgccgcaggcctggcacctcctctcgctgcccggtgccggcggtgccgggtgtcccctgcggtccaggctgcccacaagcctgtggaatgtcccctgccccgcgtcccggagccggggagccccgttgatgtagtcggcgaggtcgggcttggagcgcagggggccctggtccgcggcctgcaacacggtgctcagcacctggcgctggcgctgctgcagccgctccaggtgacggaactcggcttcgcgggcggactcatcctcaaagcgcacgtgcgacggcgaggggccccgcctcggcctgtgcccaccgctggactctccgctggaggaatcgctcgtgtgcccgttctggaggctgtctctgcaggcaggggtcgtcctggggtcccgggctgggcttctgtggccatctcggctgccctgggtaatggtgggcacgatgtcatggctggcacggaggggccgggtcctggccttcatgcgggcacgctgcagcagatgcgtggcttcctcatgcctggggctcagcacaggctccgggttgggaccaacggtcctgttctggccggagtcctgcaaggaggtgcccgaggcccagtccacatcccccactggtcgctctggtgcagctgtgtcccaggatggagtccaggcaggggttcccaccttgcgggggctctgcccagaaacgttgagcatctcctgcagcaacaggcggtttctctccacccgatcagacagggacaagacactgctcccagcgcccagagcctccaggtctccagctctccagcgctcacccagcagggccgtcctggggacaaagacctcctcggaggtcagggatgtgctatccagatctgcctctgtcaccacgccatctggaaaagggtaggaccttcctgtccttgggctgggaatgtggatgattttgttacaatgaccaggacccccaggccgtccgggagtaactccatggatcgggctctgttgcaaagagctgggccccagcagcggacctctgtcatggtcaggaagtgtccattcggcttctggaggccacgggctccccctgttgcagtactcacgtccaggggcaggcggcctgggaagcctggggcctccatccctggcgggttgctcctcattgatgctgccgtccagctgcccatcaggcaggttttgggtacgaggagccaccacagcacctggcaggaaagacccctctgatggagtcccggctctccctgccttgcctcgtctgcattggggtttcttgggggatgaccactcttgggaagcagagcagggactcactccctgtttggccactgtcatcttctccttcaaagccctcaccttggattccagcacagaggggccctggagctgtactccccataccctgggaggctggggggccatcaggctggatgttctgttttcctgagggcaaggccagggtcttggggggtgtccgttatccagctgtggctcaggaccactccactccacagctgaggtcccctccacggggctggctgttccactccctgtcttgggcccttgggggctgccgcccgcgggtttggccgccgccgcctctgtcccctccatccctcggagaggccaggccctctccagccccttctccctcccaggccagctgctgggttcggggagggacttccagccccgaatccggggccggagggagtgcggcccgcaggcctcgcccctcggggcgcggccgactgggggtccgggacggcgccgaggccgggccagctcccggctctgctggcagcccccgggccccgggtgggtctggccggcgcagcgccccacgggccgcactccctcccggcgagaggacgggaagcggggtcgggcagggagggcgctggcagggaaggaagtggcatcagctgtccgttcacggctttgccgtggaggggaagagc

SEQ ID NO: 15330 - RNA, 1511 nt, Homo sapiens
  source 1..1511: mol_type = other RNA
gctgggattacaggcatgagccactgcgcccggcctagttttgtatttttagtagagatggggtttctccgtgttggtcagactggtctcgaactcccgacctcaggtgatccgcccgcctcagcctcccaaagtgctgggataacaggcgtgagccaccgcgcccggcccctttctctttctctgtggatgttcccagcagctctctcaaaaataaaacgtgccagttcccaaaatccgcccaagaaagctgtggctcagagagggaggcactagcctaaggtgacagtgagtctgggcttagaacacagatctcctggcttcgtgtccagggaactttcttcatgcctctaattcattctctccaacaggagtttggcatgtactatgccctagagcggaggtgtgcaggacaggtgctgctgtccctgtgcacaggttaagaaacagtttaactgaatctcagggaggccaagtgactaagcaccaggacacgaaaccagaaggcagaggtctcgattttgaactcggatcatccgccagggcaacgcccggaagcctcagggcgcgcgtggctgggcgcgagctcggcgcgcagcggtgggaatcccgagcggagttggaagccgggcccgttcatttgcatgctaatacccagaatgcttttcccccgcacaccgcttctcttaatggaagcgctcagtttggaaccgtggaaagtttggaacacatacttcgctgcctctttgcaactgtgggaacttcccgcccgcacacgcggcgcctgcagcctggggctccgcgccaggcggcccaaaggcagccgccagcgcttcctgggaagacaaaccttggtgtacaactctagcgtggtagcatccccgggcgggccggggacaaagcgccgaggcctggcggcagggcccattaccagagcacccggcgtctcacagggctgcgggcgctggggatgctccgggcttggagaggcctgagggtgtccccgactcctccggcacccccacttccctgaggattgctggggcttccgggggtccctgccccgtccatcgccctcatattgtcgcctcccggagctggtgacttcacgctccccggggacaaagctcggcgtgctgtggtttgggggagaagctggacgctggcttcatctctccagctcttccgggcgcgcagcccatcagatcgatcaatgtaccgggtgcagaagcagctccggaggttcggcctgtctccggccaggaccccgggccctctctggtgtttgaagcagggaggcggtcgcaggcgacttctgggaatttcacgcatgaaagcggggctccgaagggtggacgacgcccgctcgacctgcgagtgcgcttcgcaggctggggggcccggatccgcacccctcagttcctgcccccccaccctgctagccgccactctcagcgggcaggggaggggcagtgggagctggtttgctggctcggcgcttcgtttgcatt

SEQ ID NO: 15331 - RNA, 2753 nt, Homo sapiens
  source 1..2753: mol_type = other RNA
gctgggattacaggcatgagccactgcgcccggcctatttcttttacccttggaggtagttgcacttctcacttggttcagtctcgtttgatgtcctgagctttgccataactccctgggaaactgcttatttttatactttctcttttattttagtctcttgaaatatcaaataccacaataccaaaatcagatgtacggttgcctcacataacccttgatgtttataagttgcttttgtcattgtgcggcatgcactgttatttatctaatcagcatttcagggaaacaccaagtcagaggaactttcttcctgttcctaaccgcctttgagatattacatacaggccaagtaccacaggcagggaggctttttaccgttcttacagagaggcaggtgtctctccacagtccaaagcctgaagaggccactgccacccagtaagatgattcttctgtccagctttcaagtccatccactacccctggagtaaggtgggacacaccttcaatgaacttagatcttcctcccagcctctgtccccatttctaaagtgcacaaatacatagtcccaatcctgtgacgttccttcccgcacacagacgaagatcctgctgctcttatactgtaagggtggtagacattaggcaggtctttttctctcagaaaccatgttcacagttaattaataagattatacatccataagttaaatttagaaaactgaagtcatgataagagaccacagttctcaggtaagtaaaattcctatctcaaagtagttttaaatgaatgtacggtggtttctagattaaaaaataataataattatgcaattgccaagagagtaaatttccagaggaatgggtatttttgctgtataagtattcttggagggcaaataagaccgaatctacaggccactagttttctaagtcaagtatgatcttaacagaatgccacagtaattatcctgtagttctctgcatgctctgttgattttaatacttttgataacttccattcagtagttcccttgaacatgaatcctttacaaccaaagccaggtttgtaagtttcaaggttatcgtgcaatctgaaactcggaaagatcatcacagggtccttacagctacccacataggccattccatcgttatcctggcttaatgaattatcagtccaaatgcaaagacatagccagaaacttggccttccccacaatgttgttccagatagtcatgggtgacttcttcctaagcaccccatggaatcagtgcttttagttttctcagttcacagatgaggaacctagacttagttaagtgacttctgtgaaggcatgcctgtggcaaagccaggttccaactcagcgattatgacgtcagaacagagcttttatttactttgccatagaattaacatcacggttgggaatattggatgaatcccagtgcagctaaaccaactgctgtcagcagaggtgaactgaggtaatatacaaaatcgataacacaggaaatgttctagcagctttagcaagatccagaaagcaatcaggactgaacatgcatgttgctcctttctttttcttttttttttttttttaagtaaaaacaccatttttatctctaacctcttcctcacacagaggctatagaattccccatgtaagtttttgccccatcctctctccagaccaattattgaagttagtcttcccaagatgacaactgatcaaaagattcatgtaataaaactctaatttcataataaggatttttcacaatttgaaaatgccctcaccttaagatgttgaggaacttggttcagttacttcacaggccatttactctccaactgcacagctggaattgcttccttttcaatttcagccttctgaaagatggtctttccatattgtccttaataactattttagaccctacagcctctaatattttaattaattcttactcatcctaatatactagaaaatatataaataaaaaatttaaaattgtcattgtgtcttcaagtattaaaagtaggactcagaaactgaactttaaaaaagtaatatttcaaagtgatattttcttcagcagtgatatcacaagaaacatttttaacccagattttgaagaatggatagaagtatactaatatgcttttaaaatactatttcctgctgtaattcacaaagaagagaacaaactaatcaagtaatagttctgatttatcaataatctacttaatagccttttttatagtagatctttcttatgatttctatactttatttttactaaggggctgctatttcatattttataaaacagaagactcaacagaaattaagttaaattaaattaacagaaagcctgctttttaaccacaaaactcaggtttcaaatgatttggttacatgaattttctgaccaacttaactttagctttaatagcttgttagtttcagtacttgtcttcataagacttgtccagtaaattcacatatattttgctctgctaaggagcttgtaattcattgttcgaaaccctgataattatttcaacatttgccttaatgagaataatttagcaaatataaatttatctttgtatgctaatcaaagatattataattcattgtaagaaattccaattgttaaaagctctatagacatgagtatttgggtgattagtataaatatagaataacccccaaacagccccttgatatttttaaaat

SEQ ID NO: 15332 - RNA, 542 nt, Homo sapiens
  source 1..542: mol_type = other RNA
gctgggattacaggcatgagccactgcgcccggcctcatttcttgcttttatgtttttttggcttccttttttaatttctccaagatctcttctggagttgtagaagccaaaagcttcaccaccttttcacgagatttaccacccttatccaaaaccacatcactcttcctgagttctaggaccttggaaagataccgacagagctcagcattagcctctccctctgatggaggtgctgcaatagctacatttacagcctctgctgtcaaatctgttacagcattttgtttggagccaggttttgcatggatggctatggtgacgcatcctttaggatcaactgccacaggacctaagggaggaagtggtctctctggttccttgctctggcttttacccttggtcgtcgcaccagccttcttaggcatctcggcgcaaagaagccgagcggagccccgagtattgggtgttgcccgaaggtgcctcagcccgctgcggagccgcagcatccccgcctgggaaggcgccggaagagccctct

SEQ ID NO: 15333 - RNA, 10224 nt, Homo sapiens
  source 1..10224: mol_type = other RNA
gctgggattacaggcatgagccactgcgcccggcctcttcctttaatttctgtacatgattagtagcaagacctagaccaactagaaggaagttagccacctctgaagagaacatcactaatttccttagcatggctttctgaattgaaaaggagtttgaacaagctggctgcatttttggaccaactaccgtgctgagacctttatattcaggtaatgagtatttgtgaagctcacatgaaattcctcctttaagactagaaaacaaaagttcaatccaaaccttgggatcggcagaaataaaaacagaattgtttacaagtgaatgagaaaatctattaacatcatgccagctgcatattcaccaccctccaggaatgcatgtcaatctgaatgtcatatccttagacagctataataagcgtaggtaggacagagtttgcttatcaccattaaatggtaataagtccatttcaaagggcaaatgaatgaaaaatgcacttgaaaactcattggatacactaagaaaaggttatctaaacttcattgtagacagaagacaaaagcatattttaagaaattcttccttaaaataaatatcctttattcatatttttatatatttcattgtcttggcttatgtctatgaatagatacaactttaattattcaaaggcaaacatgcctaaggaaagataaagcgttgaccgtatatcgcagtttgcccaggccagttccggtgtatgcctgggtttggaagaagatcacagactcaaggcaaatggggctggaatgagagtatggtgttgtttaagatctgttggagagggaatgaaagggactccattctttctctgtatttagaggttggatgagaactagcacagaaggccaaagcccaggctttgaattttgcccccttcacttaccagcattgtgactttgggcaagtcatgggacctctcttgggtatcagttcttttcaactcatggtggagtcttgtgcttggtacaaggatcactttattagatagttataattaagctgtttcaagaggtaaccacgtagggaacaaaagtctggaaatcttactggataaaatgagttaaagcagtggtccccaactttttggcaccaggaactggttttgtggaagacaatgtttccacggatggggtgggtaaggggaatggttttgggattaaactattccatctcagatcatcagtcatcgggcattagattctcacaagaagcagcaacctagatccctcacatgtgtagttcacaataggctttgcactcctctgagaatctaatgaaaccacagatctgacaggaggtggagctcaggcagcaatgctcactcacccaccactcacctcctgctgtgcggcccagttcctgcaggccatggacacctaccagtctgcggactgggggttggggacctctgagttaaagaaaccacggctgcctagcttcaagggataagaacaacaaatacaataacattcaaatacaagacagcctttaaagagataagagattataaatttattttataactgcaaagggcagaagtagatctcatgtggtggaatgaaaatagttctgtataaaaaactattgaataatgagatatatctagcaaatggaaggggctaatcttgaaaataatgctagtgaagacaggaagcagagaacttgacattcatgtttgtaaaaaaaaatcatgggggagatagtgggtcaagttggagggggcctgagaaaaattcccgtggaatgtgatagtcctttatttatcttccaattcccatgcacccttgtatatatcacttcttcgtgtttttgactcctaactgctacagctgatagagaattccaatctcatgctcctattgtaacgcattccccgttctctaaaaaaaaaaatctcaagaatctccaaagtggtagtagaaattattcatttttccttagacgagttgcctagtggttgacaaggggcacgtctgatctgcctttcttttctctagaacatacggaatggtttgaatatttattattgtagttaaagtaacatttaaaaagataaaagaaaatggtaagctctatagtcttgaaattctctccgatctctcttcctttgagcttgcttaacccttgaatcacaatatctgttgaatccctcaggtcatccgggaatatgaagctaatgagatgtgcagaatcctggaaggacttgggtattaaaggccttgggtatctgaagacatgggtgtgaggaaggcctgaaaaaacaaagatgagttagaagttttaaaaggagcagctatagcttcaaattctctcttcgacctgccaatcattcccacccaaccaatgtttcctctttggaaagactgaacaagattgaacctgaggcatcagacatggacgatggtgggggtaaaatgctgcacagagaacacatatataaaagaaggtatttagtgaattgtgagacatacccccgcccccacccttgtctaagccccactcctcccttcactcccagaacctggtaaccaggcttttaacctgaaagaaatgatattaagagactctggggaaactgacttggcatagagatttataggtcctgatatttgagtgtctccaaaatgaacatgtcccctgtttaccactattcaacaatacctgcctgcacagagagcttccaatcagcattttagtgcctcatcattaatttggacttataagcaaggatcaccagacacctgagaacatccttaaaacaaaacggaatcacaaagaatccagagaatcaagaggtaatccacagaatggagggaaacatcaaaatacctcttattaatatacttaagaagatgagacacccattaattgagaacagtagcttttaaaaaggaacgtttagggaagaaagagcttttggacatttaaatgtattagatcacacctggaatatcatgttcagttctaggaggaccctcccccacccccatcttaagaggggcattgagaaagtagaggttgccccgaggaagtcagaacctggatgtattcattcatgcacatacatgtgcatatggcaaacatttgtcatttgccttcataagccatcagacacagttctaggagcgaaggaaccagaaaagatccagaggaggctgagtgctcaggagttgggaaaggatggagacagatgatacaaaataaagtacagtggtgagcagtgtgtgagaggagagaccaccaaaagtgtctacaaaaagccctaaggggagcagctgaaggatgtgaaggggaggtgtgttaccaaaagaacagaagaaattagagcttttccttccttctttccctttctctttccctccctcccttccttccttcctctctctctctctctctctgtttcatatctgaaagcctattaaatagagggagagaatttgttctatataggagataaaaaaggattcagatagtgactcaaaatgggaaacaaactaagctgtttgggcaaggaacactaaattcctactcaagactggcttttgtctgaaaggtgttcttttcacatcctcttgcgtccagataaatccaaaatgtgccaaatagaaacctgctgtttctgctatagttctccactgaaccgagctagcttgataagctcttgtgtatctgttagtttattctaaaatcaatcaaacataagtagattgtatcaaagaggataatttcttaaattgagttatagaaaccagctctgttttggttaaaataaataggaaaattgttgaaatgcgatgattcctggctcttggatttaaagcatgaataccattctcgagcaagtcccacaaaattcaggcacagactaaaggagatggagaataaattttccagcaaataacaatggaaaaaacttaccctgtaactgtgctgtaacaacccccagaatcgggcttcagtcatcctgcatctcccaaatttttagcctttcgttgtacaaactgcaaataattgacaccaggctctgagtcagctttctgatcctcaccctcatggttcaaattggagtctaattataggagctactcctacacctccataggcagcttgcttgggattttttcttaaattattaatcagaggaaagataaatttgcctgttttacttatacagggatgaactgtctcctagctgatttttatttatttatgcataaaagtctattttttatggttacttacttttattatttccttccctgagtctggaggatagaatggtcagattagtgtatgtttcatacaaccctatctgtcattgcagcacagccctcatctataaatattccttaggctctggtgtataaattgcttcaattgttaaagtgtataaattgcttcaactgttaaagatgtatcttcccatattcccagtcactggaattcagagagcttaggtcataatgatatccctttaaacccaatgtgtcccaacatggactcagtgtcattttcttttcttcctctcaatggcagctcctttctgttctcagtcagttgcccaagctgtaaacctgagggaaccttggacacttccactctttctcatgggccacactgaattaatcagcaaagactcttatttacacttaccaaatgtatgtcccttctccattcccatcttcttcaccatttctcacccaaccagtgaaagagatgcctaaatgacctccaggttttctatccactatccaggttttccatcataatactggggactaagtgacaaatataatatatcccttaaaaaaacactcaatggctttgtaatatctttgttttagaggtcaaatttataacaaatggtactatgcaatgaatggcatagggttacattttggcctcacttaagtgacaattccaaatccatgtacaaccagggagttcttcactttctcatagatcctttgccaaaaattaggggaacaattttttagaaaaaaattactgaaataagcaaaagaaatttcttttctgagtcatggaagtaactaaactgagcatgaaattgttaccataaattgcactgaggaatttctattcagctcctgtttatgagtttgggggctgtgggtaagttcccattatgtgatttttctggctgcataacacaaaatactcgcaatattaatatgataaataggaacacatttagcatctcaaggagtaaaaggtaatcttcagattgagggagaatctagctaggtgatttttaggattcagaaatagataattatgttgagaacgaagttatgagtataaacaattctctcaatccgtctctttgccgattcttcctttcacctcaattgaaaattgaaaattattttagtgggagggctatagaggagtagaacatatttatcgaattctccacattttgaaatggctggttcactttcttatcaggaagagggagagatggccacattagcagcctcactccatcagttagacatatgtcaggtacctgcaatgttcttcacagatactaagcaagtacttacagataaataaatagttgtatgtatgctgagtgctgcaaaagaaaagtatctgttgtatttgaaggaaagacctgtcgtatctcaaaatgatattttgagaagctttcatttgagcagtatattggggaactcaaacaaagccttttcattttgatcatgccaaatcacctatagaattcacttatagagatgtatctatagtcatatcagaaattggctgctaaatggttacttagggtaaccaaacaagtctgagacagccatggacatgttcatgtcaggaacaaaacagaaaagtagtcacttgtagaacaaagtctagaatcaatgtaggaaaaaaaaaaaactgaatgaaactaggactagaagatttgagtttgagtcccagctttgctgcgtggccttggataaattgactagcctctgtgagcctccatattcccttagtggtcttcccattgtggctctacttacctaggaatagtggtgtattagtttgttttcatgctgctgctgaagaagcaagtcacattttgcatggatggcgtcaggcaaagaggaaacttagatattattttagctcctggctccatgatttttatataaaagaacaagacaaattcagcgaagatttaatatttgagtttgccaaggaaggttttcttacctagtggatgcagtcttaggtactatgccttaaattagaaggcacagttcctagttcctccttctgatgcaccattagctataaatcacaccaattaaactacaatttgtgcatccacactctggcactttcactcaacctgccaataaaatcttgagagaatcaccattggcagctaggccctaataatatctgaagtttccattttcccccacagagtttcacatttactctctcatgcatgatgccctttgtggctttatttttacagctaagacaggaatctaattccacttttgagataaatctcagagagaggaagtagttgtgtaggcaggttgggatatttttaaaaaactgcattggtatgaattacttttgtcaccgctttctatttatactgtacaattcagtttaccaaacatttttatctgtttcttcatttgatcttcacagcagtcttgtaatgtaagcaggaaatcagtgatgtctccattttatagacagggaatataaagcttcaggagagcttcacggtttttttttattcatttattgaacacctagtctattcctaacaatggactatgccatttacaactgctgttgcatttacctttcaaaaaatctgatcaggtaactactttttttctattctgcatatgagaaagctgagtattctctaaattgagtatcttatgcaaaatccacactaaaaatcaataataaacttatgattcaaacatgaatcagatttatctcagagccttaaaaaataataatacatcagttactcctgtcagccaaagaaaacaagctttgccaacttcaggaagtttctgtgttgactccattttgcaataagtctgataatcagagaaaatctgcctttatgaatctataaaacaaagcatgcatgaagccaaattgaaatttgatgtatgtaattttcagagttatatgcatattatatgaaatagctagttagggattcagattgttatttgcctataaaacttactttatttcacacattaaagaattcatgagtgtttggctgaaacctctgtaaagtttctccatccaagctgcaagagattgttctagtcaaaacaaatgatcccaattctatcaagcgccaatcttttagatccatcagctctctcataatcttctcaacagatcttgaggtaggtccaattcttattcctattttactcggcatgatcatgcttaattttcctgtcaatgtcctgttctggaagcaaattctttcaggttctgacttgttcaaaactatgaaagtcctgtctatacagaaggtagaatgatagaccctgaggtttgggaatagagatgagtgaggcatcccaagtctccaagtagcttacagtttgatagagggaagaccagcatgcacctgactaacacaatagatgaagggaagaagagcaagatgtcaagaggggaagggtggagaattgaggaagccttgcattctaaacaagccttatattctaaacaattgtggtgttataaccaatgtcatgatgtcatggaaacaaaatggcttcacggcgatccagggttgaatcctagctccatgttcaatgagctctgttacctagtagctctatgacttttgtgaagtcagttaacctctctgaacctctgtttcctcatctgtaaaataatatatctacctcagaactttcttaggaaaaataatgtatttttaaaagtatgtagtacagatcctagctcattgcaggtgctcagtaaatgtgaattccacattggatgatataaaaattgaagcatttgaaaatttcattcaaatgttctcctgaggcttggaatcaagacagtgttatgaatttgactgaaaaatgttccaaagggacaggcatagatatgagtaaaacatttgaggaagagagaattaatatttaatggatatggtagtgttaggtttttctgttttaacttgttgaaaaatacaatttcaggacttctataaaacatacttatatttcacaatttgtgtagcaggtttcctgtttacttctagagcatttctaactatgaacttgtttatctccaagaagttggagacagagctctgccgccacagatgcaccatttatatttataaacccagatcttactagttttactatgtgaaatttcttgtgtttatgtttagttttcaaagaaaagtagcaaagagacagataagcacctctgacacaggatttacattgagatgactgtcaaagtaggaaagatgaaaacaggatagattccaattaaggcaaatgcagtataaatcattcattttggggaattttaacaccatagaatgtcatgcagtcaaaacatttcgaaagcatggcagaaaacattttgggtatctaataagccatactgtaaggcaaatataatttattattaaggcaagtattctattgtgttacaaaaaatgaggcagctacaagagcctaacaaagtgttgattgtatatagatgaagtgtcagagaattgtttccaatgtatgacatgattgagatggagagatcctggagaacaataaaaataacagaagaatttggaagtggtagttatttgacggaaataaagccttggaattagaatatttagttttgaaaaaagtagcactaggggagatgcatgttcatctttcttattgcaaaaacataaaaatgaaaatggacaatttcagtacctggagccattttataactgaattcatctaggtattctactccctcatttattttttattcactcaaaaaaaagtttattgagcatctcagacactatgttaggaaaaggaagttccaagaagaatgaaaaatatttcctgccctcagagggctcagtctaatggaagatgaacaactgtacaaataactgcaagttggtgtgatgaatgcaatgaagtagcaaagtgattaaatgagggttgggacttgcacagagttagatgtttaagaaggggcagctggaaggtgggatctcctgcttttatcatgggtagtaaagtcatcaaaggtataaaggagagtgtcccatctctccagatgggagatttagtggtacttagagatgacatgtagtatttatcaagtggcaatgtaaagcatggatcagaaaaagttaagagttcttgatctgtgttccagacaaggcccttttcttctctgggaaatgctattagaggctgtatgatttttgtgcaaaggtttgaccagtagtcccacttctggtgctctgctaacctgctgccaacattcacatatacaccaagatccctgtttgtgatagcaaaaagctggacaagcctaaatatctaatgataagggagttgttaaatacagtctaaactatggaatagactattaagagtattaagaaacatgatatttatgtatttggtagaaggcaggaaaatatccaaattacactattaaaaaggggggaaaagtcttaatacaataaatagctatggtcttgtttgtatggttatgtgtgtatgtacacacagctacccacaaacacacacatacatatccggcacacaaccatacatgtaccactagggtaagctgtagggaaagagagcagtgagagagaaggtaagggaaggcagaagagacgagagcctctcaatttttatcctgtgtttttctatatctttcaaaattttcaacatccatagacttcattttgtaatttaaaacagaaatgagataatgcccatgaagcattgagcatattgtctgccatgtggccagcaataaatgttaattgactcttccaaggtggcaagaaaatacgacttgctcaaaatgatttaaatctgcatacagtatcgtatctttatttttccttaattttaaataaagacagggtctcactt

SEQ ID NO: 15334 - RNA, 4501 nt, Homo sapiens
  source 1..4501: mol_type = other RNA
gctgggattacaggcatgagccactgcgcccggcctgaactatttcaatcctaaaattggtatgtccttttacagtccttcctggtgtcttcttccttattataatagtaccactggttgtcaagtagccttatcttatatctctgtaagtattatttaaaatgaaattgaaatatcatttattttagccagaaaagaaaatggaatggctaatttggtgaatccactccctgttgatacactaagctgctgacccctggagctcagaggctgaaggcaaggctgtgaagctatgaggtaggcgtggaggtgagggctcagtcacagtggaccttgcccttggccaccccaaagctagacaagtctccattgcaaagagtctggagtggtgaatgaggcccgttttccaagtcattttggtcaccttggtcacccttggtcaccttcatcatgtactttcgaaaggccttttgaataatagcagcacctctttcctcttcctttctcttggtggtggtgactatgggttcatacaacttcttgagaggattggcttccatgaacttctcttccatcattgctttcatactatctaggccatcagagccaccgagtaccctagcggtgaaggcgaaaagaatatccatgcagtggaggcgatcttcactcaccatgggcaagtccattactagaaattgatatttatttggctttgcgacacgcaaaggctcaggcaaggcatcagcaaagtcagaaagggcagaatatttgataaattgtgttgcttctgggtcaaacttttcccacacttcataaaatatgtcaaagtcatcttcacccaaagggtcctcactttcttcagtggctgtattgaagttctctaaaatcacagcaatgtacatgttgacaacaatgagaaaggagatgataatgtaactgacaaagtaggatgtggctatgccagggaggtggcagttttctgaggaagagttacatgattcttttgatcgcagcatggggctgagcagggaatcccaacctgctgatgtgcttatctggaagagacagagcatgctgctggcaaaagtcttgaagttgaatatgtcatcgattccagactctggattcactttggaaaaccagttcatacccagaatggcatagataaacataatcagaaagagtagaagaccaatgttgaacagagaaggaagcgacatcatcagagcaaagaggagagtcctgattcctcgtgcagcccggacaagcctcaggattcggccaatccgagccaagcggacaattctgaagagcgtcggagggaaaggaatgtgctcctgattttccaaggtagaaatcattgtactaacaatggaaagaagcacgaccacacagtcaaataaattccagccattggtgaagtagtattgcctcaaagcaaagattttgatgagacattctaacgtaaagatgaccacaaagacccagttgagatggtcaaggatggatttcatggctttgggttggttgtatgattcagccatcatgctaatcatgtttaggataatgagacttatgatgatgatgtcaaagatctggcttgtgactatgtcgaacacgagaccttgacatttgttcagaggccgtggaatgggtttttgaggttttttggatcctaattttttcattgcattatagtatttcttctgttcttctgtcataaaaatgtcttggccacctaactttttctgctgttggttgaagttgtcaatgataacgccaatgaagagattcagagtgaagaatgagccaaagatgataaagactacgaagtaaatgtaaccgagtgaattgctctcaaactctggctgttgttctttctctgtggaatcaacagctgcatatataatatccatccagcccttaaatgttgccacttgcagcagagcgaggtaagcatttcccacattgtcaaagttgactttctggttgatccaagagaaattgccactttcacattgacttttatttgtaatgatggtataatttataactgagtctgttccattaatgcatttcccaaattttccagaaaagaagtatactcccagaatacaaaatacgagccagaaaatgaggcagacaagcaaaacattcagaatggcaggtatggcacctatgagagcattgaccaccaccttcattccttcaaactgggacagcgcacgaagaggcctcagtgctcgtagagtccggaaggacttcaattccattaagttaatgagggtggtcacagagacaatcacaatgatgaaatcaaggcagcaccaggcactggtgaaatactttccaaatccgaaggctacccattttagtaccatctccaggataaaaatatgtgtaaaaataatgtcagtacaatttagtaattcttggattttgggttggttctcaaggtgaacatcttcaaatatcagtgccccactgctcagcagaatcacaaagataataaagctctcaaaccagctgtgtttcactatttggtagcaggttttccgcaggttccaccaaatgacccagggaggctttctcttgtccacgctacagcatggaaagcagcaaccaaagcctttgggcaaacatctctctggttgctttttgggaaccatctcaggtaaccatccaaagccatcctgaagatcaatggtgctacattctgatagtatactggtaacatcagacttctttcggggatcctgtatggtcagatgaggctcatcttcagagaacatgtcaatttccacactttgaactctctggctcgtgggcttcttgttctcctgatggagctcataggcctgttgttcaggctcaggttgtgtgatgcgctgtgcattatcttcaccagaaaattcaacgtcatcttcctcctccgcaagtggtgccaaccaagtccaatcatgcctgacgcccagggtctttggtacagaggttagtataccaagctcctcctgggtctctgagccccttttcatctccatgaccaggggaatgatgtctttgctttgtgcagcacagcctcctgccacctctttttgctgtggtaagttttgcttcctgcaccacttgtgacagaaatgctcaagagtgtgtctcacaaaacaaaaagcccggcggaatcgatccagtgctaactggactttagttttcctggcctctccttctaagtttccatttctttcctcattgctaaaggaattgagcagtaaggcaatgaagaggttgagcaccacaagttttcctatcaccgtgatcaatatgaagacaataacacacaatgatgatgatgcattcgcttcttgcatacattcccacatattttcgatccattccccgcagaggatgcggaataccactaggaaggagtgccagaaatcccccatgtgccagtgccgtaaacatgagactgtcgggcctgtcgggttacagagttttggactcttttgggaattgaagctacggccaaaaagctgcatgccaactactgagaaaataaagatcacaatgaccaggaccacagtcaggcttccaagggctccgacagagttgccgattatcttaattagtgtgttcaaagttggccaggatttggctaacttgaagaccctgagcactctgaaggaacgcaagaatggccagcttctcttttgaagtacacagttcattacatctgcaaaactcagaagagcaacaatgctgtcaaaaatgttccagcctcggcgaaagtagtggtagggatcgagcgcaatgatttttaggcacatttctgctataaaaatgctagtgaaaaccaaattccctatattcaacatcttctcaaaactggcctccatcttgtgatgctccatggccaagaagacagtgttgatgatgatgcagatggtgatggccagctcagtaaacgggtcagtcatcacagttctcaggaccttcttaacgcacagccactgggggcaacagttccacacgaggtacttggatgccaggttttctccacaagggagacaaggctcttgtgatttttcttgttccttcatggtgatggtgaggatgctgacagcactcagtgctctctgcctttggagaggatctccatgctcatcaaagtggtccagtgatagattctgggacagtcgtttggtttgctctaggagctgtggctcgtctttacagcatgccaaatattcagttttcttatttcatgtttaacaaataagagaaatctggtttgatcattcatatttcctatgcatgcacatttctagagtcctacctacagacattttactttctctgtgtttcattcactgccaacaaagagcaaacaaaattttacaaaaactagtaagcaatggttccgggtatgaaagcaatacaaaatccaatttgtaaacaatgtttaaaggtaagaagtggagtataaatttagaaaggtggactg

SEQ ID NO: 15335 - RNA, 5549 nt, Homo sapiens
  source 1..5549: mol_type = other RNA
gctgggattacaggcatgagccactgcgcccggcctgaactatttcaatcctaaaattggtatgtccttttacagtccttcctggtgtcttcttccttattataatagtaccactggttgtcaagtagccttatcttatatctctgtaagtattatttaaaatgaaattgaaatatcatttattttagccagaaaagaaaatggaatggctaatttggtgaatccactccctgttgatacactaagctgctgacccctggagctcagaggctgaaggcaaggctgtgaagctatgaggtaggcgtggaggtgagggctcagtcacagtggaccttgcccttggccaccccaaagctagacaagtctccattgcaaagagtctggagtggtgaatgaggcccgttttccaagtcattttggtcaccttggtcacccttggtcaccttcatcatgtactttcgaaaggccttttgaataatagcagcacctctttcctcttcctttctcttggtggtggtgactatgggttcatacaacttcttgagaggattggcttccatgaacttctcttccatcattgctttcatactatctaggccatcagagccaccgagtaccctagcggtgaaggcgaaaagaatatccatgcagtggaggcgatcttcactcaccatgggcaagtccattactagaaattgatatttatttggctttgcgacacgcaaaggctcaggcaaggcatcagcaaagtcagaaagggcagaatatttgataaattgtgttgcttctgggtcaaacttttcccacacttcataaaatatgtcaaagtcatcttcacccaaagggtcctcactttcttcagtggctgtattgaagttctctaaaatcacagcaatgtacatgttgacaacaatgagaaaggagatgataatgtaactgacaaagtaggatgtggctatgccagggaggtggcagttttctgaggaagagttacatgattcttttgatcgcagcatggggctgagcagggaatcccaacctgctgatgtgcttatctggaagagacagagcatgctgctggcaaaagtcttgaagttgaatatgtcatcgattccagactctggattcactttggaaaaccagttcatacccagaatggcatagataaacataatcagaaagagtagaagaccaatgttgaacagagaaggaagcgacatcatcagagcaaagaggagagtcctgattcctcgtgcagcccggacaagcctcaggattcggccaatccgagccaagcggacaattctgaagagcgtcggagggaaaggaatgtgctcctgattttccaaggtagaaatcattgtactaacaatggaaagaagcacgaccacacagtcaaataaattccagccattggtgaagtagtattgcctcaaagcaaagattttgatgagacattctaacgtaaagatgaccacaaagacccagttgagatggtcaaggatggatttcatggctttgggttggttgtatgattcagccatcatgctaatcatgtttaggataatgagacttatgatgatgatgtcaaagatctggcttgtgactatgtcgaacacgagaccttgacatttgttcagaggccgtggaatgggtttttgaggttttttggatcctaattttttcattgcattatagtatttcttctgttcttctgtcataaaaatgtcttggccacctaactttttctgctgttggttgaagttgtcaatgataacgccaatgaagagattcagagtgaagaatgagccaaagatgataaagactacgaagtaaatgtaaccgagtgaattgctctcaaactctggctgttgttctttctctgtggaatcaacagctgcatatataatatccatccagcccttaaatgttgccacttgcagcagagcgaggtaagcatttcccacattgtcaaagttgactttctggttgatccaagagaaattgccactttcacattgacttttatttgtaatgatggtataatttataactgagtctgttccattaatgcatttcccaaattttccagaaaagaagtatactcccagaatacaaaatacgagccagaaaatgaggcagacaagcaaaacattcagaatggcaggtatggcacctatgagagcattgaccaccaccttcattccttcaaactgggacagcgcacgaagaggcctcagtgctcgtagagtccggaaggacttcaattccattaagttaatgagggtggtcacagagacaatcacaatgatgaaatcaaggcagcaccaggcactggtgaaatactttccaaatccgaaggctacccattttagtaccatctccaggataaaaatatgtgtaaaaataatgtcagtacaatttagtaattcttggattttgggttggttctcaaggtgaacatcttcaaatatcagtgccccactgctcagcagaatcacaaagataataaagctctcaaaccagctgtgtttcactatttggtagcaggttttccgcaggttccaccaaatgacccagggaggctttctcttgtccacgctacagcatggaaagcagcaaccaaagcctttgggcaaacatctctctggttgctttttgggaaccatctcaggtaaccatccaaagccatcctgaagatcaatggtgctacattctgatagtatactggtaacatcagacttctttcggggatcctgtatggtcagatgaggctcatcttcagagaacatgtcaatttccacactttgaactctctggctcgtgggcttcttgttctcctgatggagctcataggcctgttgttcaggctcaggttgtgtgatgcgctgtgcattatcttcaccagaaaattcaacgtcatcttcctcctccgcaagtggtgccaaccaagtccaatcatgcctgacgcccagggtctttggtacagaggttagtataccaagctcctcctgggtctctgagccccttttcatctccatgaccaggggaatgatgtctttgctttgtgcagcacagcctcctgccacctctttttgctgtggtaagttttgcttcctgcaccacttgtgacagaaatgctcaagagtgtgtctcacaaaacaaaaagcccggcggaatcgatccagtgctaactggactttagttttcctggcctctccttctaagtttccatttctttcctcattgctaaaggaattgagcagtaaggcaatgaagaggttgagcaccacaagttttcctatcaccgtgatcaatatgaagacaataacacacaatgatgatgatgcattcgcttcttgcatacattcccacatattttcgatccattccccgcagaggatgcggaataccactaggaaggagtgccagaaatcccccatgtgccagtgccgtaaacatgagactgtcgggcctgtcgggttacagagttttggactcttttgggaattgaagctacggccaaaaagctgcatgccaactactgagaaaataaagatcacaatgaccaggaccacagtcaggcttccaagggctccgacagagttgccgattatcttaattagtgtgttcaaagttggccaggatttggctaacttgaagaccctgagcactctgaaggaacgcaagaatggccagcttctcttttgaagtacacagttcattacatctgcaaaactcagaagagcaacaatgctgtcaaaaatgttccagcctcggcgaaagtagtggtagggatcgagcgcaatgatttttaggcacatttctgctataaaaatgctagtgaaaaccaaattccctatattcaacatcttctcaaaactggcctccatcttgtgatgctccatggccaagaagacagtgttgatgatgatgcagatggtgatggccagctcagtaaacgggtcagtcatcacagttctcaggaccttcttaacgcacagccactgggggcaacagttccacacgaggtacttggatgccaggttttctccacaagggagacaaggctcttgtgatttttcttgttccttcatggtgatggtgaggatgctgacagcactcagtgctctctgcctttggagaggatctccatgctcatcaaagtggtccagtgatagattctgggacagtcgtttggtttgctctaggagctgtggctttttttggcaatcttcatcagaatctgacccaggaggctggtctttcccagactctctcaaaaagaaggacttccttttcttattaccaaagagctttctcttttttggggtaaaatatgatgtttcaagggaagtaagtgaacttctgtcaattcccatggcaaccagagcctccttttcctcctttaacagctgctgggcttcctgaaacatcttttccttggcctctatctctgcagctacattcttgttctgctcctcatatgccatggtaacaacagccagggttaagttaatcaggtagaaggagcccaggaaaatgaccacaatgaagaagaagactgagtagagcccagtagtacgcagggtctgttgataaagcttctcccaggaatcttgggtcatcagccggaacatggcaagaaaagaccagccaaagttgtcaaaattcgtataattatagtcaggattaattttggtgtgcttacattcatattgtatggaacaggcactgttacccatccagatgccacacattttgaattcaggtgaattttctttcttttcaaagcaatggtcataagcttccgggttactgatatttttacagtccctcgagatgcatttcaggttcagacttcccatgaagagctgctgacctaccagggcaaagatgctgaggcaaaagaaggtgaggataatcacgttgaccagcttcttcacagagcgtagcaaggcccccacgatgaccttcagacgtgaaactactgaaattgctttcaaagctctgaacacacggaaggtacgcaggggcaatagtttgatggtgattcctggaatatatgacacaatcgctattccaatgacaatggagtccagccagttccatggatctcgaaggaaagaaaactcatccagaatgaaacctcttgccaatattttaatcaaagcttcaaaaatataaatcccagtgaagacacactctgcaatgtcagtattgttactgttgctgtttttagcaggccctgtagccatgaacacgcagttgatgataacggtgccgataatgaacatgctgaacaatgaatggactgagactctaatggctaaacttctgattgaattgaaaggcccaaaaatgaacaaggcatgcttggcactgaagcggtagattgtcctctttctgtttaacaccataaatgtccaatgggatactccagaagaatcagagatggaaaacacaggaccttatgatttcggtagaatgggtccaagtcttccagaggctttcctatgagctcacgaggaatgtcgccatagagcttg

SEQ ID NO: 15336 - RNA, 6180 nt, Homo sapiens
  source 1..6180: mol_type = other RNA
gctgggattacaggcatgagccactgcgcccggcctgaactatttcaatcctaaaattggtatgtccttttacagtccttcctggtgtcttcttccttattataatagtaccactggttgtcaagtagccttatcttatatctctgtaagtattatttaaaatgaaattgaaatatcatttattttagccagaaaagaaaatggaatggctaatttggtgaatccactccctgttgatacactaagctgctgacccctggagctcagaggctgaaggcaaggctgtgaagctatgaggtaggcgtggaggtgagggctcagtcacagtggaccttgcccttggccaccccaaagctagacaagtctccattgcaaagagtctggagtggtgaatgaggcccgttttccaagtcattttggtcaccttggtcacccttggtcaccttcatcatgtactttcgaaaggccttttgaataatagcagcacctctttcctcttcctttctcttggtggtggtgactatgggttcatacaacttcttgagaggattggcttccatgaacttctcttccatcattgctttcatactatctaggccatcagagccaccgagtaccctagcggtgaaggcgaaaagaatatccatgcagtggaggcgatcttcactcaccatgggcaagtccattactagaaattgatatttatttggctttgcgacacgcaaaggctcaggcaaggcatcagcaaagtcagaaagggcagaatatttgataaattgtgttgcttctgggtcaaacttttcccacacttcataaaatatgtcaaagtcatcttcacccaaagggtcctcactttcttcagtggctgtattgaagttctctaaaatcacagcaatgtacatgttgacaacaatgagaaaggagatgataatgtaactgacaaagtaggatgtggctatgccagggaggtggcagttttctgaggaagagttacatgattcttttgatcgcagcatggggctgagcagggaatcccaacctgctgatgtgcttatctggaagagacagagcatgctgctggcaaaagtcttgaagttgaatatgtcatcgattccagactctggattcactttggaaaaccagttcatacccagaatggcatagataaacataatcagaaagagtagaagaccaatgttgaacagagaaggaagcgacatcatcagagcaaagaggagagtcctgattcctcgtgcagcccggacaagcctcaggattcggccaatccgagccaagcggacaattctgaagagcgtcggagggaaaggaatgtgctcctgattttccaaggtagaaatcattgtactaacaatggaaagaagcacgaccacacagtcaaataaattccagccattggtgaagtagtattgcctcaaagcaaagattttgatgagacattctaacgtaaagatgaccacaaagacccagttgagatggtcaaggatggatttcatggctttgggttggttgtatgattcagccatcatgctaatcatgtttaggataatgagacttatgatgatgatgtcaaagatctggcttgtgactatgtcgaacacgagaccttgacatttgttcagaggccgtggaatgggtttttgaggttttttggatcctaattttttcattgcattatagtatttcttctgttcttctgtcataaaaatgtcttggccacctaactttttctgctgttggttgaagttgtcaatgataacgccaatgaagagattcagagtgaagaatgagccaaagatgataaagactacgaagtaaatgtaaccgagtgaattgctctcaaactctggctgttgttctttctctgtggaatcaacagctgcatatataatatccatccagcccttaaatgttgccacttgcagcagagcgaggtaagcatttcccacattgtcaaagttgactttctggttgatccaagagaaattgccactttcacattgacttttatttgtaatgatggtataatttataactgagtctgttccattaatgcatttcccaaattttccagaaaagaagtatactcccagaatacaaaatacgagccagaaaatgaggcagacaagcaaaacattcagaatggcaggtatggcacctatgagagcattgaccaccaccttcattccttcaaactgggacagcgcacgaagaggcctcagtgctcgtagagtccggaaggacttcaattccattaagttaatgagggtggtcacagagacaatcacaatgatgaaatcaaggcagcaccaggcactggtgaaatactttccaaatccgaaggctacccattttagtaccatctccaggataaaaatatgtgtaaaaataatgtcagtacaatttagtaattcttggattttgggttggttctcaaggtgaacatcttcaaatatcagtgccccactgctcagcagaatcacaaagataataaagctctcaaaccagctgtgtttcactatttggtagcaggttttccgcaggttccaccaaatgacccagggaggctttctcttgtccacgctacagcatggaaagcagcaaccaaagcctttgggcaaacatctctctggttgctttttgggaaccatctcaggtaaccatccaaagccatcctgaagatcaatggtgctacattctgatagtatactggtaacatcagacttctttcggggatcctgtatggtcagatgaggctcatcttcagagaacatgtcaatttccacactttgaactctctggctcgtgggcttcttgttctcctgatggagctcataggcctgttgttcaggctcaggttgtgtgatgcgctgtgcattatcttcaccagaaaattcaacgtcatcttcctcctccgcaagtggtgccaaccaagtccaatcatgcctgacgcccagggtctttggtacagaggttagtataccaagctcctcctgggtctctgagccccttttcatctccatgaccaggggaatgatgtctttgctttgtgcagcacagcctcctgccacctctttttgctgtggtaagttttgcttcctgcaccacttgtgacagaaatgctcaagagtgtgtctcacaaaacaaaaagcccggcggaatcgatccagtgctaactggactttagttttcctggcctctccttctaagtttccatttctttcctcattgctaaaggaattgagcagtaaggcaatgaagaggttgagcaccacaagttttcctatcaccgtgatcaatatgaagacaataacacacaatgatgatgatgcattcgcttcttgcatacattcccacatattttcgatccattccccgcagaggatgcggaataccactaggaaggagtgccagaaatcccccatgtgccagtgccgtaaacatgagactgtcgggcctgtcgggttacagagttttggactcttttgggaattgaagctacggccaaaaagctgcatgccaactactgagaaaataaagatcacaatgaccaggaccacagtcaggcttccaagggctccgacagagttgccgattatcttaattagtgtgttcaaagttggccaggatttggctaacttgaagaccctgagcactctgaaggaacgcaagaatggccagcttctcttttgaagtacacagttcattacatctgcaaaactcagaagagcaacaatgctgtcaaaaatgttccagcctcggcgaaagtagtggtagggatcgagcgcaatgatttttaggcacatttctgctataaaaatgctagtgaaaaccaaattccctatattcaacatcttctcaaaactggcctccatcttgtgatgctccatggccaagaagacagtgttgatgatgatgcagatggtgatggccagctcagtaaacgggtcagtcatcacagttctcaggaccttcttaacgcacagccactgggggcaacagttccacacgaggtacttggatgccaggttttctccacaagggagacaaggctcttgtgatttttcttgttccttcatggtgatggtgaggatgctgacagcactcagtgctctctgcctttggagaggatctccatgctcatcaaagtggtccagtgatagattctgggacagtcgtttggtttgctctaggagctgtggctttttttggcaatcttcatcagaatctgacccaggaggctggtctttcccagactctctcaaaaagaaggacttccttttcttattaccaaagagctttctcttttttggggtaaaatatgatgtttcaagggaagtaagtgaacttctgtcaattcccatggcaaccagagcctccttttcctcctttaacagctgctgggcttcctgaaacatcttttccttggcctctatctctgcagctacattcttgttctgctcctcatatgccatggtaacaacagccagggttaagttaatcaggtagaaggagcccaggaaaatgaccacaatgaagaagaagactgagtagagcccagtagtacgcagggtctgttgataaagcttctcccaggaatcttgggtcatcagccggaacatggcaagaaaagaccagccaaagttgtcaaaattcgtataattatagtcaggattaattttggtgtgcttacattcatattgtatggaacaggcactgttacccatccagatgccacacattttgaattcaggtgaattttctttcttttcaaagcaatggtcataagcttccgggttactgatatttttacagtccctcgagatgcatttcaggttcagacttcccatgaagagctgctgacctaccagggcaaagatgctgaggcaaaagaaggtgaggataatcacgttgaccagcttcttcacagagcgtagcaaggcccccacgatgaccttcagacgtgaaactactgaaattgctttcaaagctctgaacacacggaaggtacgcaggggcaatagtttgatggtgattcctggaatatatgacacaatcgctattccaatgacaatggagtccagccagttccatggatctcgaaggaaagaaaactcatccagaatgaaacctcttgccaatattttaatcaaagcttcaaaaatataaatcccagtgaagacacactctgcaatgtcagtattgttactgttgctgtttttagcaggccctgtagccatgaacacgcagttgatgataacggtgccgataatgaacatgctgaacaatgaatggactgagactctaatggctaaacttctgattgaattgaaaggcccaaaaatgaacaaggcatgcttggcactgaagcggtagattgtcctctttctgtttaacaccataaatgtcttatgatttcggtagaatgggtccaagtcttccagaggctttcctatgagctcacgaggaatgtcgccatagagcttgggcaacttcctggaggcctttaggtcaagctgaggccgaggctggggtacttctcctgtctggtctttagacttctttttctccttttggatggcaatccgcttctcaattgcagccagagagtcggaagtgaaggggcggaaattccgctcatctggaaagattactgggtagcatctgtcatccatcttcacccgagattcctggcttgagcagatgagaggacagtgtggccactcactgagacagagagtgcaagaaaaggagggcactgcgagggaataaatttggtttgcaacacacgaagctgaagctgcctggggaacctgacttcttggtaaggtggctccagacagcaatcccagcgatacttcttgaagctctccacagagcaagtctctcagcagagttcgagcttctgctcctggcagctgcctggagcccttctgggaggagcggcttggaggcgctcccctctggtaaacaagatgccaactctagggtacggtggaaagacatactggatactttcactgtgttcagcaaatggattgaacatggagccaaaaacatgcgaagcactgggacaatctcatcacatggctaccggccacacagcaactaacagcaccgaggaaacacaacagcctgtttaccttcagccccgccactaac

SEQ ID NO: 15337 - RNA, 6344 nt, Homo sapiens
  source 1..6344: mol_type = other RNA
gctgggattacaggcatgagccactgcgcccggcctgaactatttcaatcctaaaattggtatgtccttttacagtccttcctggtgtcttcttccttattataatagtaccactggttgtcaagtagccttatcttatatctctgtaagtattatttaaaatgaaattgaaatatcatttattttagccagaaaagaaaatggaatggctaatttggtgaatccactccctgttgatacactaagctgctgacccctggagctcagaggctgaaggcaaggctgtgaagctatgaggtaggcgtggaggtgagggctcagtcacagtggaccttgcccttggccaccccaaagctagacaagtctccattgcaaagagtctggagtggtgaatgaggcccgttttccaagtcattttggtcaccttggtcacccttggtcaccttcatcatgtactttcgaaaggccttttgaataatagcagcacctctttcctcttcctttctcttggtggtggtgactatgggttcatacaacttcttgagaggattggcttccatgaacttctcttccatcattgctttcatactatctaggccatcagagccaccgagtaccctagcggtgaaggcgaaaagaatatccatgcagtggaggcgatcttcactcaccatgggcaagtccattactagaaattgatatttatttggctttgcgacacgcaaaggctcaggcaaggcatcagcaaagtcagaaagggcagaatatttgataaattgtgttgcttctgggtcaaacttttcccacacttcataaaatatgtcaaagtcatcttcacccaaagggtcctcactttcttcagtggctgtattgaagttctctaaaatcacagcaatgtacatgttgacaacaatgagaaaggagatgataatgtaactgacaaagtaggatgtggctatgccagggaggtggcagttttctgaggaagagttacatgattcttttgatcgcagcatggggctgagcagggaatcccaacctgctgatgtgcttatctggaagagacagagcatgctgctggcaaaagtcttgaagttgaatatgtcatcgattccagactctggattcactttggaaaaccagttcatacccagaatggcatagataaacataatcagaaagagtagaagaccaatgttgaacagagaaggaagcgacatcatcagagcaaagaggagagtcctgattcctcgtgcagcccggacaagcctcaggattcggccaatccgagccaagcggacaattctgaagagcgtcggagggaaaggaatgtgctcctgattttccaaggtagaaatcattgtactaacaatggaaagaagcacgaccacacagtcaaataaattccagccattggtgaagtagtattgcctcaaagcaaagattttgatgagacattctaacgtaaagatgaccacaaagacccagttgagatggtcaaggatggatttcatggctttgggttggttgtatgattcagccatcatgctaatcatgtttaggataatgagacttatgatgatgatgtcaaagatctggcttgtgactatgtcgaacacgagaccttgacatttgttcagaggccgtggaatgggtttttgaggttttttggatcctaattttttcattgcattatagtatttcttctgttcttctgtcataaaaatgtcttggccacctaactttttctgctgttggttgaagttgtcaatgataacgccaatgaagagattcagagtgaagaatgagccaaagatgataaagactacgaagtaaatgtaaccgagtgaattgctctcaaactctggctgttgttctttctctgtggaatcaacagctgcatatataatatccatccagcccttaaatgttgccacttgcagcagagcgaggtaagcatttcccacattgtcaaagttgactttctggttgatccaagagaaattgccactttcacattgacttttatttgtaatgatggtataatttataactgagtctgttccattaatgcatttcccaaattttccagaaaagaagtatactcccagaatacaaaatacgagccagaaaatgaggcagacaagcaaaacattcagaatggcaggtatggcacctatgagagcattgaccaccaccttcattccttcaaactgggacagcgcacgaagaggcctcagtgctcgtagagtccggaaggacttcaattccattaagttaatgagggtggtcacagagacaatcacaatgatgaaatcaaggcagcaccaggcactggtgaaatactttccaaatccgaaggctacccattttagtaccatctccaggataaaaatatgtgtaaaaataatgtcagtacaatttagtaattcttggattttgggttggttctcaaggtgaacatcttcaaatatcagtgccccactgctcagcagaatcacaaagataataaagctctcaaaccagctgtgtttcactatttggtagcaggttttccgcaggttccaccaaatgacccagggaggctttctcttgtccacgctacagcatggaaagcagcaaccaaagcctttgggcaaacatctctctggttgctttttgggaaccatctcaggtaaccatccaaagccatcctgaagatcaatggtgctacattctgatagtatactggtaacatcagacttctttcggggatcctgtatggtcagatgaggctcatcttcagagaacatgtcaatttccacactttgaactctctggctcgtgggcttcttgttctcctgatggagctcataggcctgttgttcaggctcaggttgtgtgatgcgctgtgcattatcttcaccagaaaattcaacgtcatcttcctcctccgcaagtggtgccaaccaagtccaatcatgcctgacgcccagggtctttggtacagaggttagtataccaagctcctcctgggtctctgagccccttttcatctccatgaccaggggaatgatgtctttgctttgtgcagcacagcctcctgccacctctttttgctgtggtaagttttgcttcctgcaccacttgtgacagaaatgctcaagagtgtgtctcacaaaacaaaaagcccggcggaatcgatccagtgctaactggactttagttttcctggcctctccttctaagtttccatttctttcctcattgctaaaggaattgagcagtaaggcaatgaagaggttgagcaccacaagttttcctatcaccgtgatcaatatgaagacaataacacacaatgatgatgatgcattcgcttcttgcatacattcccacatattttcgatccattccccgcagaggatgcggaataccactaggaaggagtgccagaaatcccccatgtgccagtgccgtaaacatgagactgtcgggcctgtcgggttacagagttttggactcttttgggaattgaagctacggccaaaaagctgcatgccaactactgagaaaataaagatcacaatgaccaggaccacagtcaggcttccaagggctccgacagagttgccgattatcttaattagtgtgttcaaagttggccaggatttggctaacttgaagaccctgagcactctgaaggaacgcaagaatggccagcttctcttttgaagtacacagttcattacatctgcaaaactcagaagagcaacaatgctgtcaaaaatgttccagcctcggcgaaagtagtggtagggatcgagcgcaatgatttttaggcacatttctgctataaaaatgctagtgaaaaccaaattccctatattcaacatcttctcaaaactggcctccatcttgtgatgctccatggccaagaagacagtgttgatgatgatgcagatggtgatggccagctcagtaaacgggtcagtcatcacagttctcaggaccttcttaacgcacagccactgggggcaacagttccacacgaggtacttggatgccaggttttctccacaagggagacaaggctcttgtgatttttcttgttccttcatggtgatggtgaggatgctgacagcactcagtgctctctgcctttggagaggatctccatgctcatcaaagtggtccagtgatagattctgggacagtcgtttggtttgctctaggagctgtggctttttttggcaatcttcatcagaatctgacccaggaggctggtctttcccagactctctcaaaaagaaggacttccttttcttattaccaaagagctttctcttttttggggtaaaatatgatgtttcaagggaagtaagtgaacttctgtcaattcccatggcaaccagagcctccttttcctcctttaacagctgctgggcttcctgaaacatcttttccttggcctctatctctgcagctacattcttgttctgctcctcatatgccatggtaacaacagccagggttaagttaatcaggtagaaggagcccaggaaaatgaccacaatgaagaagaagactgagtagagcccagtagtacgcagggtctgttgataaagcttctcccaggaatcttgggtcatcagccggaacatggcaagaaaagaccagccaaagttgtcaaaattcgtataattatagtcaggattaattttggtgtgcttacattcatattgtatggaacaggcactgttacccatccagatgccacacattttgaattcaggtgaattttctttcttttcaaagcaatggtcataagcttccgggttactgatatttttacagtccctcgagatgcatttcaggttcagacttcccatgaagagctgctgacctaccagggcaaagatgctgaggcaaaagaaggtgaggataatcacgttgaccagcttcttcacagagcgtagcaaggcccccacgatgaccttcagacgtgaaactactgaaattgctttcaaagctctgaacacacggaaggtacgcaggggcaatagtttgatggtgattcctggaatatatgacacaatcgctattccaatgacaatggagtccagccagttccatggatctcgaaggaaagaaaactcatccagaatgaaacctcttgccaatattttaatcaaagcttcaaaaatataaatcccagtgaagacacactctgcaatgtcagtattgttactgttgctgtttttagcaggccctgtagccatgaacacgcagttgatgataacggtgccgataatgaacatgctgaacaatgaatggactgagactctaatggctaaacttctgattgaattgaaaggcccaaaaatgaacaaggcatgcttggcactgaagcggtagattgtcctctttctgtttaacaccataaatgtcttatgatttcggtagaatgggtccaagtcttccagaggctttcctatgagctcacgaggaatgtcgccatagagcttgggcaacttcctggaggcctttaggtcaagctgaggccgaggctggggtacttctcctgtctggtctttagacttctttttctccttttggatggcaatccgcttctcaattgcagccagagagtcggaagtgaaggggcggaaattccgctcatctggaaagattactgggtagcatctgtcatccatcttcacccgagattcctggcttgagcagatgagaggacagtgtggccactcactgagacagagagtgcaagaaaaggagggcactgcgagggaataaatttggtttgcaacacacgaagctgaagctgcctggggaacctttattatgggtccaaatatagtacagttcttggttccggaaaatagtagctgacttcttggtaaggtggctccagacagcaatcccagcgatacttcttgaagctctccacagagcaagtctctcagcagagttcgagcttctgctcctggcagctgcctggagcccttctgggaggagcggcttggaggagggtgtccatttggcatctcctcctttctcttctcttgtgccattaaccttggggttcagacctgagatcattggttgtttctgttcagaagttgcagcgctggtgaaattcagctgctttccagaacgttgccatcaaggctgtttggcccaacccaaaaattcgaggcaagtttctgagggtttttgttgttgttgtttgcaaggttgcaggtcgtcagtcctccctagaatggcttcctgacttcactttagagatctgaaccagagggacatcattttgtgtatcagtttcacataacaaaggaaattaacatttg

SEQ ID NO: 15338 - RNA, 5892 nt, Homo sapiens
  source 1..5892: mol_type = other RNA
gctgggattacaggcatgagccactgcgcccggcctgaactatttcaatcctaaaattggtatgtccttttacagtccttcctggtgtcttcttccttattataatagtaccactggttgtcaagtagccttatcttatatctctgtaagtattatttaaaatgaaattgaaatatcatttattttagccagaaaagaaaatggaatggctaatttggtgaatccactccctgttgatacactaagctgctgacccctggagctcagaggctgaaggcaaggctgtgaagctatgaggtaggcgtggaggtgagggctcagtcacagtggaccttgcccttggccaccccaaagctagacaagtctccattgcaaagagtctggagtggtgaatgaggcccgttttccaagtcattttggtcaccttggtcacccttggtcaccttcatcatgtactttcgaaaggccttttgaataatagcagcacctctttcctcttcctttctcttggtggtggtgactatgggttcatacaacttcttgagaggattggcttccatgaacttctcttccatcattgctttcatactatctaggccatcagagccaccgagtaccctagcggtgaaggcgaaaagaatatccatgcagtggaggcgatcttcactcaccatgggcaagtccattactagaaattgatatttatttggctttgcgacacgcaaaggctcaggcaaggcatcagcaaagtcagaaagggcagaatatttgataaattgtgttgcttctgggtcaaacttttcccacacttcataaaatatgtcaaagtcatcttcacccaaagggtcctcactttcttcagtggctgtattgaagttctctaaaatcacagcaatgtacatgttgacaacaatgagaaaggagatgataatgtaactgacaaagtaggatgtggctatgccagggaggtggcagttttctgaggaagagttacatgattcttttgatcgcagcatggggctgagcagggaatcccaacctgctgatgtgcttatctggaagagacagagcatgctgctggcaaaagtcttgaagttgaatatgtcatcgattccagactctggattcactttggaaaaccagttcatacccagaatggcatagataaacataatcagaaagagtagaagaccaatgttgaacagagaaggaagcgacatcatcagagcaaagaggagagtcctgattcctcgtgcagcccggacaagcctcaggattcggccaatccgagccaagcggacaattctgaagagcgtcggagggaaaggaatgtgctcctgattttccaaggtagaaatcattgtactaacaatggaaagaagcacgaccacacagtcaaataaattccagccattggtgaagtagtattgcctcaaagcaaagattttgatgagacattctaacgtaaagatgaccacaaagacccagttgagatggtcaaggatggatttcatggctttgggttggttgtatgattcagccatcatgctaatcatgtttaggataatgagacttatgatgatgatgtcaaagatctggcttgtgactatgtcgaacacgagaccttgacatttgttcagaggccgtggaatgggtttttgaggttttttggatcctaattttttcattgcattatagtatttcttctgttcttctgtcataaaaatgtcttggccacctaactttttctgctgttggttgaagttgtcaatgataacgccaatgaagagattcagagtgaagaatgagccaaagatgataaagactacgaagtaaatgtaaccgagtgaattgctctcaaactctggctgttgttctttctctgtggaatcaacagctgcatatataatatccatccagcccttaaatgttgccacttgcagcagagcgaggtaagcatttcccacattgtcaaagttgactttctggttgatccaagagaaattgccactttcacattgacttttatttgtaatgatggtataatttataactgagtctgttccattaatgcatttcccaaattttccagaaaagaagtatactcccagaatacaaaatacgagccagaaaatgaggcagacaagcaaaacattcagaatggcaggtatggcacctatgagagcattgaccaccaccttcattccttcaaactgggacagcgcacgaagaggcctcagtgctcgtagagtccggaaggacttcaattccattaagttaatgagggtggtcacagagacaatcacaatgatgaaatcaaggcagcaccaggcactggtgaaatactttccaaatccgaaggctacccattttagtaccatctccaggataaaaatatgtgtaaaaataatgtcagtacaatttagtaattcttggattttgggttggttctcaaggtgaacatcttcaaatatcagtgccccactgctcagcagaatcacaaagataataaagctctcaaaccagctgtgtttcactatttggtagcaggttttccgcaggttccaccaaatgacccagggaggctttctcttgtccacgctacagcatggaaagcagcaaccaaagcctttgggcaaacatctctctggttgctttttgggaaccatctcaggtaaccatccaaagccatcctgaagatcaatggtgctacattctgatagtatactggtaacatcagacttctttcggggatcctgtatggtcagatgaggctcatcttcagagaacatgtcaatttccacactttgaactctctggctcgtgggcttcttgttctcctgatggagctcataggcctgttgttcaggctcaggttgtgtgatgcgctgtgcattatcttcaccagaaaattcaacgtcatcttcctcctccgcaagtggtgccaaccaagtccaatcatgcctgacgcccagggtctttggtacagaggttagtataccaagctcctcctgggtctctgagccccttttcatctccatgaccaggggaatgatgtctttgctttgtgcagcacagcctcctgccacctctttttgctgtggtaagttttgcttcctgcaccacttgtgacagaaatgctcaagagtgtgtctcacaaaacaaaaagcccggcggaatcgatccagtgctaactggactttagttttcctggcctctccttctaagtttccatttctttcctcattgctaaaggaattgagcagtaaggcaatgaagaggttgagcaccacaagttttcctatcaccgtgatcaatatgaagacaataacacacaatgatgatgatgcattcgcttcttgcatacattcccacatattttcgatccattccccgcagaggatgcggaataccactaggaaggagtgccagaaatcccccatgtgccagtgccgtaaacatgagactgtcgggcctgtcgggttacagagttttggactcttttgggaattgaagctacggccaaaaagctgcatgccaactactgagaaaataaagatcacaatgaccaggaccacagtcaggcttccaagggctccgacagagttgccgattatcttaattagtgtgttcaaagttggccaggatttggctaacttgaagaccctgagcactctgaaggaacgcaagaatggccagcttctcttttgaagtacacagttcattacatctgcaaaactcagaagagcaacaatgctgtcaaaaatgttccagcctcggcgaaagtagtggtagggatcgagcgcaatgatttttaggcacatttctgctataaaaatgctagtgaaaaccaaattccctatattcaacatcttctcaaaactggcctccatcttgtgatgctccatggccaagaagacagtgttgatgatgatgcagatggtgatggccagctcagtaaacgggtcagtcatcacagttctcaggaccttcttaacgcacagccactgggggcaacagttccacacgaggtacttggatgccaggttttctccacaagggagacaaggctcttgtgatttttcttgttccttcatggtgatggtgaggatgctgacagcactcagtgctctctgcctttggagaggatctccatgctcatcaaagtggtccagtgatagattctgggacagtcgtttggtttgctctaggagctgtggctttttttggcaatcttcatcagaatctgacccaggaggctggtctttcccagactctctcaaaaagaaggacttccttttcttattaccaaagagctttctcttttttggggtaaaatatgatgtttcaagggaagtaagtgaacttctgtcaattcccatggcaaccagagcctccttttcctcctttaacagctgctgggcttcctgaaacatcttttccttggcctctatctctgcagctacattcttgttctgctcctcatatgccatggtaacaacagccagggttaagttaatcaggtagaaggagcccaggaaaatgaccacaatgaagaagaagactgagtagagcccagtagtacgcagggtctgttgataaagcttctcccaggaatcttgggtcatcagccggaacatggcaagaaaagaccagccaaagttgtcaaaattcgtataattatagtcaggattaattttggtgtgcttacattcatattgtatggaacaggcactgttacccatccagatgccacacattttgaattcaggtgaattttctttcttttcaaagcaatggtcataagcttccgggttactgatatttttacagtccctcgagatgcatttcaggttcagacttcccatgaagagctgctgacctaccagggcaaagatgctgaggcaaaagaaggtgaggataatcacgttgaccagcttcttcacagagcgtagcaaggcccccacgatgaccttcagacgtgaaactactgaaattgctttcaaagctctgaacacacggaaggtacgcaggggcaatagtttgatggtgattcctggaatatatgacacaatcgctattccaatgacaatggagtccagccagttccatggatctcgaaggaaagaaaactcatccagaatgaaacctcttgccaatattttaatcaaagcttcaaaaatataaatcccagtgaagacacactctgcaatgtcagtattgttactgttgctgtttttagcaggccctgtagccatgaacacgcagttgatgataacggtgccgataatgaacatgctgaacaatgaatggactgagactctaatggctaaacttctgattgaattgaaaggcccaaaaatgaacaaggcatgcttggcactgaagcggtagattgtcctctttctgtttaacaccataaatgtcttatgatttcggtagaatgggtccaagtcttccagaggctttcctatgagctcacgaggaatgtcgccatagagcttgggcaacttcctggaggcctttaggtcaagctgaggccgaggctggggtacttctcctgtctggtctttagacttctttttctccttttggatggcaatccgcttctcaattgcagccagagagtcggaagtgaaggggcggaaattccgctcatctggaaagattactgggtagcatctgtcatccatcttcaccctcaggacagagacaagccacagatcctcagaaaggcctcaggaggcgggaataaaacagcctgccctaggattccagtcttaaaggatggtgtcataaggatctacaaaagctgagctgaggtcaggggccttgggagctgattggctgtgaagatcagaagagatgaccaccactgtgggtatagcagga

SEQ ID NO: 15339 - RNA, 6023 nt, Homo sapiens
  source 1..6023: mol_type = other RNA
gctgggattacaggcatgagccactgcgcccggcctgaactatttcaatcctaaaattggtatgtccttttacagtccttcctggtgtcttcttccttattataatagtaccactggttgtcaagtagccttatcttatatctctgtaagtattatttaaaatgaaattgaaatatcatttattttagccagaaaagaaaatggaatggctaatttggtgaatccactccctgttgatacactaagctgctgacccctggagctcagaggctgaaggcaaggctgtgaagctatgaggtaggcgtggaggtgagggctcagtcacagtggaccttgcccttggccaccccaaagctagacaagtctccattgcaaagagtctggagtggtgaatgaggcccgttttccaagtcattttggtcaccttggtcacccttggtcaccttcatcatgtactttcgaaaggccttttgaataatagcagcacctctttcctcttcctttctcttggtggtggtgactatgggttcatacaacttcttgagaggattggcttccatgaacttctcttccatcattgctttcatactatctaggccatcagagccaccgagtaccctagcggtgaaggcgaaaagaatatccatgcagtggaggcgatcttcactcaccatgggcaagtccattactagaaattgatatttatttggctttgcgacacgcaaaggctcaggcaaggcatcagcaaagtcagaaagggcagaatatttgataaattgtgttgcttctgggtcaaacttttcccacacttcataaaatatgtcaaagtcatcttcacccaaagggtcctcactttcttcagtggctgtattgaagttctctaaaatcacagcaatgtacatgttgacaacaatgagaaaggagatgataatgtaactgacaaagtaggatgtggctatgccagggaggtggcagttttctgaggaagagttacatgattcttttgatcgcagcatggggctgagcagggaatcccaacctgctgatgtgcttatctggaagagacagagcatgctgctggcaaaagtcttgaagttgaatatgtcatcgattccagactctggattcactttggaaaaccagttcatacccagaatggcatagataaacataatcagaaagagtagaagaccaatgttgaacagagaaggaagcgacatcatcagagcaaagaggagagtcctgattcctcgtgcagcccggacaagcctcaggattcggccaatccgagccaagcggacaattctgaagagcgtcggagggaaaggaatgtgctcctgattttccaaggtagaaatcattgtactaacaatggaaagaagcacgaccacacagtcaaataaattccagccattggtgaagtagtattgcctcaaagcaaagattttgatgagacattctaacgtaaagatgaccacaaagacccagttgagatggtcaaggatggatttcatggctttgggttggttgtatgattcagccatcatgctaatcatgtttaggataatgagacttatgatgatgatgtcaaagatctggcttgtgactatgtcgaacacgagaccttgacatttgttcagaggccgtggaatgggtttttgaggttttttggatcctaattttttcattgcattatagtatttcttctgttcttctgtcataaaaatgtcttggccacctaactttttctgctgttggttgaagttgtcaatgataacgccaatgaagagattcagagtgaagaatgagccaaagatgataaagactacgaagtaaatgtaaccgagtgaattgctctcaaactctggctgttgttctttctctgtggaatcaacagctgcatatataatatccatccagcccttaaatgttgccacttgcagcagagcgaggtaagcatttcccacattgtcaaagttgactttctggttgatccaagagaaattgccactttcacattgacttttatttgtaatgatggtataatttataactgagtctgttccattaatgcatttcccaaattttccagaaaagaagtatactcccagaatacaaaatacgagccagaaaatgaggcagacaagcaaaacattcagaatggcaggtatggcacctatgagagcattgaccaccaccttcattccttcaaactgggacagcgcacgaagaggcctcagtgctcgtagagtccggaaggacttcaattccattaagttaatgagggtggtcacagagacaatcacaatgatgaaatcaaggcagcaccaggcactggtgaaatactttccaaatccgaaggctacccattttagtaccatctccaggataaaaatatgtgtaaaaataatgtcagtacaatttagtaattcttggattttgggttggttctcaaggtgaacatcttcaaatatcagtgccccactgctcagcagaatcacaaagataataaagctctcaaaccagctgtgtttcactatttggtagcaggttttccgcaggttccaccaaatgacccagggaggctttctcttgtccacgctacagcatggaaagcagcaaccaaagcctttgggcaaacatctctctggttgctttttgggaaccatctcaggtaaccatccaaagccatcctgaagatcaatggtgctacattctgatagtatactggtaacatcagacttctttcggggatcctgtatggtcagatgaggctcatcttcagagaacatgtcaatttccacactttgaactctctggctcgtgggcttcttgttctcctgatggagctcataggcctgttgttcaggctcaggttgtgtgatgcgctgtgcattatcttcaccagaaaattcaacgtcatcttcctcctccgcaagtggtgccaaccaagtccaatcatgcctgacgcccagggtctttggtacagaggttagtataccaagctcctcctgggtctctgagccccttttcatctccatgaccaggggaatgatgtctttgctttgtgcagcacagcctcctgccacctctttttgctgtggtaagttttgcttcctgcaccacttgtgacagaaatgctcaagagtgtgtctcacaaaacaaaaagcccggcggaatcgatccagtgctaactggactttagttttcctggcctctccttctaagtttccatttctttcctcattgctaaaggaattgagcagtaaggcaatgaagaggttgagcaccacaagttttcctatcaccgtgatcaatatgaagacaataacacacaatgatgatgatgcattcgcttcttgcatacattcccacatattttcgatccattccccgcagaggatgcggaataccactaggaaggagtgccagaaatcccccatgtgccagtgccgtaaacatgagactgtcgggcctgtcgggttacagagttttggactcttttgggaattgaagctacggccaaaaagctgcatgccaactactgagaaaataaagatcacaatgaccaggaccacagtcaggcttccaagggctccgacagagttgccgattatcttaattagtgtgttcaaagttggccaggatttggctaacttgaagaccctgagcactctgaaggaacgcaagaatggccagcttctcttttgaagtacacagttcattacatctgcaaaactcagaagagcaacaatgctgtcaaaaatgttccagcctcggcgaaagtagtggtagggatcgagcgcaatgatttttaggcacatttctgctataaaaatgctagtgaaaaccaaattccctatattcaacatcttctcaaaactggcctccatcttgtgatgctccatggccaagaagacagtgttgatgatgatgcagatggtgatggccagctcagtaaacgggtcagtcatcacagttctcaggaccttcttaacgcacagccactgggggcaacagttccacacgaggtacttggatgccaggttttctccacaagggagacaaggctcttgtgatttttcttgttccttcatggtgatggtgaggatgctgacagcactcagtgctctctgcctttggagaggatctccatgctcatcaaagtggtccagtgatagattctgggacagtcgtttggtttgctctaggagctgtggctttttttggcaatcttcatcagaatctgacccaggaggctggtctttcccagactctctcaaaaagaaggacttccttttcttattaccaaagagctttctcttttttggggtaaaatatgatgtttcaagggaagtaagtgaacttctgtcaattcccatggcaaccagagcctccttttcctcctttaacagctgctgggcttcctgaaacatcttttccttggcctctatctctgcagctacattcttgttctgctcctcatatgccatggtaacaacagccagggttaagttaatcaggtagaaggagcccaggaaaatgaccacaatgaagaagaagactgagtagagcccagtagtacgcagggtctgttgataaagcttctcccaggaatcttgggtcatcagccggaacatggcaagaaaagaccagccaaagttgtcaaaattcgtataattatagtcaggattaattttggtgtgcttacattcatattgtatggaacaggcactgttacccatccagatgccacacattttgaattcaggtgaattttctttcttttcaaagcaatggtcataagcttccgggttactgatatttttacagtccctcgagatgcatttcaggttcagacttcccatgaagagctgctgacctaccagggcaaagatgctgaggcaaaagaaggtgaggataatcacgttgaccagcttcttcacagagcgtagcaaggcccccacgatgaccttcagacgtgaaactactgaaattgctttcaaagctctgaacacacggaaggtacgcaggggcaatagtttgatggtgattcctggaatatatgacacaatcgctattccaatgacaatggagtccagccagttccatggatctcgaaggaaagaaaactcatccagaatgaaacctcttgccaatattttaatcaaagcttcaaaaatataaatcccagtgaagacacactctgcaatgtcagtattgttactgttgctgtttttagcaggccctgtagccatgaacacgcagttgatgataacggtgccgataatgaacatgctgaacaatgaatggactgagactctaatggctaaacttctgattgaattgaaaggcccaaaaatgaacaaggcatgcttggcactgaagcggtagattgtcctctttctgtttaacaccataaatgtcttatgatttcggtagaatgggtccaagtcttccagaggctttcctatgagctcacgaggaatgtcgccatagagcttgggcaacttcctggaggcctttaggtcaagctgaggccgaggctggggtacttctcctgtctggtctttagacttctttttctccttttggatggcaatccgcttctcaattgcagccagagagtcggaagtgaaggggcggaaattccgctcatctggaaagattactgggtagcatctgtcatccatcttcaccctcaggacagagacaagccacagatcctcagaaaggcctcaggaggcgggaataaaacagcctgccctaggattccagtcttaaaggatggtgtcataaggatctacaaaagctgagctgaggtcaggggccttgggagctgattggctgtgaagatcagaagagatgaccaccactgtgggtatagcaggaacttttggcatagacaaaaccaaagcagggcatcattcctggaggacctgacttcttggtaaggtggctccagacagcaatcccagcgatacttcttgaagctctccacagagcaagtctctcagcagagt

SEQ ID NO: 15340 - RNA, 5117 nt, Homo sapiens
  source 1..5117: mol_type = other RNA
gctgggattacaggcatgagccactgcgcccggcctgaactatttcaatcctaaaattggtatgtccttttacagtccttcctggtgtcttcttccttattataatagtaccactggttgtcaagtagccttatcttatatctctgtaagtattatttaaaatgaaattgaaatatcatttattttagccagaaaagaaaatggaatggctaatttggtgaatccactccctgttgatacactaagctgctgacccctggagctcagaggctgaaggcaaggctgtgaagctatgaggtaggcgtggaggtgagggctcagtcacagtggaccttgcccttggccaccccaaagctagacaagtctccattgcaaagagtctggagtggtgaatgaggcccgttttccaagtcattttggtcaccttggtcacccttggtcaccttcatcatgtactttcgaaaggccttttgaataatagcagcacctctttcctcttcctttctcttggtggtggtgactatgggttcatacaacttcttgagaggattggcttccatgaacttctcttccatcattgctttcatactatctaggccatcagagccaccgagtaccctagcggtgaaggcgaaaagaatatccatgcagtggaggcgatcttcactcaccatgggcaagtccattactagaaattgatatttatttggctttgcgacacgcaaaggctcaggcaaggcatcagcaaagtcagaaagggcagaatatttgataaattgtgttgcttctgggtcaaacttttcccacacttcataaaatatgtcaaagtcatcttcacccaaagggtcctcactttcttcagtggctgtattgaagttctctaaaatcacagcaatgtacatgttgacaacaatgagaaaggagatgataatgtaactgacaaagtaggatgtggctatgccagggaggtggcagttttctgaggaagagttacatgattcttttgatcgcagcatggggctgagcagggaatcccaacctgctgatgtgcttatctggaagagacagagcatgctgctggcaaaagtcttgaagttgaatatgtcatcgattccagactctggattcactttggaaaaccagttcatacccagaatggcatagataaacataatcagaaagagtagaagaccaatgttgaacagagaaggaagcgacatcatcagagcaaagaggagagtcctgattcctcgtgcagcccggacaagcctcaggattcggccaatccgagccaagcggacaattctgaagagcgtcggagggaaaggaatgtgctcctgattttccaaggtagaaatcattgtactaacaatggaaagaagcacgaccacacagtcaaataaattccagccattggtgaagtagtattgcctcaaagcaaagattttgatgagacattctaacgtaaagatgaccacaaagacccagttgagatggtcaaggatggatttcatggctttgggttggttgtatgattcagccatcatgctaatcatgtttaggataatgagacttatgatgatgatgtcaaagatctggcttgtgactatgtcgaacacgagaccttgacatttgttcagaggccgtggaatgggtttttgaggttttttggatcctaattttttcattgcattatagtatttcttctgttcttctgtcataaaaatgtcttggccacctaactttttctgctgttggttgaagttgtcaatgataacgccaatgaagagattcagagtgaagaatgagccaaagatgataaagactacgaagtaaatgtaaccgagtgaattgctctcaaactctggctgttgttctttctctgtggaatcaacagctgcatatataatatccatccagcccttaaatgttgccacttgcagcagagcgaggtaagcatttcccacattgtcaaagttgactttctggttgatccaagagaaattgccactttcacattgacttttatttgtaatgatggtataatttataactgagtctgttccattaatgcatttcccaaattttccagaaaagaagtatactcccagaatacaaaatacgagccagaaaatgaggcagacaagcaaaacattcagaatggcaggtatggcacctatgagagcattgaccaccaccttcattccttcaaactgggacagcgcacgaagaggcctcagtgctcgtagagtccggaaggacttcaattccattaagttaatgagggtggtcacagagacaatcacaatgatgaaatcaaggcagcaccaggcactggtgaaatactttccaaatccgaaggctacccattttagtaccatctccaggataaaaatatgtgtaaaaataatgtcagtacaatttagtaattcttggattttgggttggttctcaaggtgaacatcttcaaatatcagtgccccactgctcagcagaatcacaaagataataaagctctcaaaccagctgtgtttcactatttggtagcaggttttccgcaggttccaccaaatgacccagggaggctttctcttgtccacgctacagcatggaaagcagcaaccaaagcctttgggcaaacatctctctggttgctttttgggaaccatctcaggtaaccatccaaagccatcctgaagatcaatggtgctacattctgatagtatactggtaacatcagacttctttcggggatcctgtatggtcagatgaggctcatcttcagagaacatgtcaatttccacactttgaactctctggctcgtgggcttcttgttctcctgatggagctcataggcctgttgttcaggctcaggttgtgtgatgcgctgtgcattatcttcaccagaaaattcaacgtcatcttcctcctccgcaagtggtgccaaccaagtccaatcatgcctgacgcccagggtctttggtacagaggttagtataccaagctcctcctgggtctctgagccccttttcatctccatgaccaggggaatgatgtctttgctttgtgcagcacagcctcctgccacctctttttgctgtggtaagttttgcttcctgcaccacttgtgacagaaatgctcaagagtgtgtctcacaaaacaaaaagcccggcggaatcgatccagtgctaactggactttagttttcctggcctctccttctaagtttccatttctttcctcattgctaaaggaattgagcagtaaggcaatgaagaggttgagcaccacaagttttcctatcaccgtgatcaatatgaagacaataacacacaatgatgatgatgcattcgcttcttgcatacattcccacatattttcgatccattccccgcagaggatgcggaataccactaggaaggagtgccagaaatcccccatgtgccagtgccgtaaacatgagactgtcgggcctgtcgggttacagagttttggactcttttgggaattgaagctacggccaaaaagctgcatgccaactactgagaaaataaagatcacaatgaccaggaccacagtcaggcttccaagggctccgacagagttgccgattatcttaattagtgtgttcaaagttggccaggatttggctaacttgaagaccctgagcactctgaaggaacgcaagaatggccagcttctcttttgaagtacacagttcattacatctgcaaaactcagaagagcaacaatgctgtcaaaaatgttccagcctcggcgaaagtagtggtagggatcgagcgcaatgatttttaggcacatttctgctataaaaatgctagtgaaaaccaaattccctatattcaacatcttctcaaaactggcctccatcttgtgatgctccatggccaagaagacagtgttgatgatgatgcagatggtgatggccagctcagtaaacgggtcagtcatcacagttctcaggaccttcttaacgcacagccactgggggcaacagttccacacgaggtacttggatgccaggttttctccacaagggagacaaggctcttgtgatttttcttgttccttcatggtgatggtgaggatgctgacagcactcagtgctctctgcctttggagaggatctccatgctcatcaaagtggtccagtgatagattctgggacagtcgtttggtttgctctaggagctgtggctttttttggcaatcttcatcagaatctgacccaggaggctggtctttcccagactctctcaaaaagaaggacttccttttcttattaccaaagagctttctcttttttggggtaaaatatgatgtttcaagggaagtaagtgaacttctgtcaattcccatggcaaccagagcctccttttcctcctttaacagctgctgggcttcctgaaacatcttttccttggcctctatctctgcagctacattcttgttctgctcctcatatgccatggtaacaacagccagggttaagttaatcaggtagaaggagcccaggaaaatgaccacaatgaagaagaagactgagtagagcccagtagtacgcagggtctgttgataaagcttctcccaggaatcttgggtcatcagccggaacatggcaagaaaagaccagccaaagttgtcaaaattcgtataattatagtcaggattaattttggtgtgcttacattcatattgtatggaacaggcactgttacccatccagatgccacacattttgaattcaggtgaattttctttcttttcaaagcaatggtcataagcttccgggttactgatatttttacagtccctcgagatgcatttcaggttcagacttcccatgaagagctgctgacctaccagggcaaagatggtgaaactactgaaattgctttcaaagctctgaacacacggaaggtacgcaggggcaatagtttgatggtgattcctggaatatatgacacaatcgctattccaatgacaatggagtccagccagttccatggatctcgaaggaaagaaaactcatccagaatgaaacctcttgccaatattttaatcaaagcttcaaaaatataaatcccagtgaag

SEQ ID NO: 15341 - RNA, 5825 nt, Homo sapiens
  source 1..5825: mol_type = other RNA
gctgggattacaggcatgagccactgcgcccggcctgaactatttcaatcctaaaattggtatgtccttttacagtccttcctggtgtcttcttccttattataatagtaccactggttgtcaagtagccttatcttatatctctgtaagtattatttaaaatgaaattgaaatatcatttattttagccagaaaagaaaatggaatggctaatttggtgaatccactccctgttgatacactaagctgctgacccctggagctcagaggctgaaggcaaggctgtgaagctatgaggtaggcgtggaggtgagggctcagtcacagtggaccttgcccttggccaccccaaagctagacaagtctccattgcaaagagtctggagtggtgaatgaggcccgttttccaagtcattttggtcaccttggtcacccttggtcaccttcatcatgtactttcgaaaggccttttgaataatagcagcacctctttcctcttcctttctcttggtggtggtgactatgggttcatacaacttcttgagaggattggcttccatgaacttctcttccatcattgctttcatactatctaggccatcagagccaccgagtaccctagcggtgaaggcgaaaagaatatccatgcagtggaggcgatcttcactcaccatgggcaagtccattactagaaattgatatttatttggctttgcgacacgcaaaggctcaggcaaggcatcagcaaagtcagaaagggcagaatatttgataaattgtgttgcttctgggtcaaacttttcccacacttcataaaatatgtcaaagtcatcttcacccaaagggtcctcactttcttcagtggctgtattgaagttctctaaaatcacagcaatgtacatgttgacaacaatgagaaaggagatgataatgtaactgacaaagtaggatgtggctatgccagggaggtggcagttttctgaggaagagttacatgattcttttgatcgcagcatggggctgagcagggaatcccaacctgctgatgtgcttatctggaagagacagagcatgctgctggcaaaagtcttgaagttgaatatgtcatcgattccagactctggattcactttggaaaaccagttcatacccagaatggcatagataaacataatcagaaagagtagaagaccaatgttgaacagagaaggaagcgacatcatcagagcaaagaggagagtcctgattcctcgtgcagcccggacaagcctcaggattcggccaatccgagccaagcggacaattctgaagagcgtcggagggaaaggaatgtgctcctgattttccaaggtagaaatcattgtactaacaatggaaagaagcacgaccacacagtcaaataaattccagccattggtgaagtagtattgcctcaaagcaaagattttgatgagacattctaacgtaaagatgaccacaaagacccagttgagatggtcaaggatggatttcatggctttgggttggttgtatgattcagccatcatgctaatcatgtttaggataatgagacttatgatgatgatgtcaaagatctggcttgtgactatgtcgaacacgagaccttgacatttgttcagaggccgtggaatgggtttttgaggttttttggatcctaattttttcattgcattatagtatttcttctgttcttctgtcataaaaatgtcttggccacctaactttttctgctgttggttgaagttgtcaatgataacgccaatgaagagattcagagtgaagaatgagccaaagatgataaagactacgaagtaaatgtaaccgagtgaattgctctcaaactctggctgttgttctttctctgtggaatcaacagctgcatatataatatccatccagcccttaaatgttgccacttgcagcagagcgaggtaagcatttcccacattgtcaaagttgactttctggttgatccaagagaaattgccactttcacattgacttttatttgtaatgatggtataatttataactgagtctgttccattaatgcatttcccaaattttccagaaaagaagtatactcccagaatacaaaatacgagccagaaaatgaggcagacaagcaaaacattcagaatggcaggtatggcacctatgagagcattgaccaccaccttcattccttcaaactgggacagcgcacgaagaggcctcagtgctcgtagagtccggaaggacttcaattccattaagttaatgagggtggtcacagagacaatcacaatgatgaaatcaaggcagcaccaggcactggtgaaatactttccaaatccgaaggctacccattttagtaccatctccaggataaaaatatgtgtaaaaataatgtcagtacaatttagtaattcttggattttgggttggttctcaaggtgaacatcttcaaatatcagtgccccactgctcagcagaatcacaaagataataaagctctcaaaccagctgtgtttcactatttggtagcaggttttccgcaggttccaccaaatgacccagggaggctttctcttgtccacgctacagcatggaaagcagcaaccaaagcctttgggcaaacatctctctggttgctttttgggaaccatctcaggtaaccatccaaagccatcctgaagatcaatggtgctacattctgatagtatactggtaacatcagacttctttcggggatcctgtatggtcagatgaggctcatcttcagagaacatgtcaatttccacactttgaactctctggctcgtgggcttcttgttctcctgatggagctcataggcctgttgttcaggctcaggttgtgtgatgcgctgtgcattatcttcaccagaaaattcaacgtcatcttcctcctccgcaagtggtgccaaccaagtccaatcatgcctgacgcccagggtctttggtacagaggttagtataccaagctcctcctgggtctctgagccccttttcatctccatgaccaggggaatgatgtctttgctttgtgcagcacagcctcctgccacctctttttgctgtggtaagttttgcttcctgcaccacttgtgacagaaatgctcaagagtgtgtctcacaaaacaaaaagcccggcggaatcgatccagtgctaactggactttagttttcctggcctctccttctaagtttccatttctttcctcattgctaaaggaattgagcagtaaggcaatgaagaggttgagcaccacaagttttcctatcaccgtgatcaatatgaagacaataacacacaatgatgatgatgcattcgcttcttgcatacattcccacatattttcgatccattccccgcagaggatgcggaataccactaggaaggagtgccagaaatcccccatgtgccagtgccgtaaacatgagactgtcgggcctgtcgggttacagagttttggactcttttgggaattgaagctacggccaaaaagctgcatgccaactactgagaaaataaagatcacaatgaccaggaccacagtcaggcttccaagggctccgacagagttgccgattatcttaattagtgtgttcaaagttggccaggatttggctaacttgaagaccctgagcactctgaaggaacgcaagaatggccagcttctcttttgaagtacacagttcattacatctgcaaaactcagaagagcaacaatgctgtcaaaaatgttccagcctcggcgaaagtagtggtagggatcgagcgcaatgatttttaggcacatttctgctataaaaatgctagtgaaaaccaaattccctatattcaacatcttctcaaaactggcctccatcttgtgatgctccatggccaagaagacagtgttgatgatgatgcagatggtgatggccagctcagtaaacgggtcagtcatcacagttctcaggaccttcttaacgcacagccactgggggcaacagttccacacgaggtacttggatgccaggttttctccacaagggagacaaggctcttgtgatttttcttgttccttcatggtgatggtgaggatgctgacagcactcagtgctctctgcctttggagaggatctccatgctcatcaaagtggtccagtgatagattctgggacagtcgtttggtttgctctaggagctgtggctttttttggcaatcttcatcagaatctgacccaggaggctggtctttcccagactctctcaaaaagaaggacttccttttcttattaccaaagagctttctcttttttggggtaaaatatgatgtttcaagggaagtaagtgaacttctgtcaattcccatggcaaccagagcctgttgataaagcttctcccaggaatcttgggtcatcagccggaacatggcaagaaaagaccagccaaagttgtcaaaattcgtataattatagtcaggattaattttggtgtgcttacattcatattgtatggaacaggcactgttacccatccagatgccacacattttgaattcaggtgaattttctttcttttcaaagcaatggtcataagcttccgggttactgatatttttacagtccctcgagatgcatttcaggttcagacttcccatgaagagctgctgacctaccagggcaaagatgctgaggcaaaagaaggtgaggataatcacgttgaccagcttcttcacagagcgtagcaaggcccccacgatgaccttcagacgtgaaactactgaaattgctttcaaagctctgaacacacggaaggtacgcaggggcaatagtttgatggtgattcctggaatatatgacacaatcgctattccaatgacaatggagtccagccagttccatggatctcgaaggaaagaaaactcatccagaatgaaacctcttgccaatattttaatcaaagcttcaaaaatataaatcccagtgaagacacactctgcaatgtcagtattgttactgttgctgtttttagcaggccctgtagccatgaacacgcagttgatgataacggtgccgataatgaacatgctgaacaatgaatggactgagactctaatggctaaacttctgattgaattgaaaggcccaaaaatgaacaaggcatgcttggcactgaagcggtagattgtcctctttctgtttaacaccataaatgtcttatgatttcggtagaatgggtccaagtcttccagaggctttcctatgagctcacgaggaatgtcgccatagagcttgggcaacttcctggaggcctttaggtcaagctgaggccgaggctggggtacttctcctgtctggtctttagacttctttttctccttttggatggcaatccgcttctcaattgcagccagagagtcggaagtgaaggggcggaaattccgctcatctggaaagattactgggtagcatctgtcatccatcttcacccgagattcctggcttgagcagatgagaggacagtgtggccactcactgagacagagagtgcaagaaaaggagggcactgcgagggaataaatttggtttgcaacacacgaagctgaagctgcctggggaacctttattatgggtccaaatatagtacagttcttggttccggaaaatagtagctgacttcttggtaaggtggctccagacagcaatcccagcgatacttcttgaagctctccacagagcaagtctctcagcagagttcgagcttctgctcctggcagctgcctggagcccttctgggaggagcggcttggagg

SEQ ID NO: 15342 - RNA, 9804 nt, Homo sapiens
  source 1..9804: mol_type = other RNA
gctgggattacaggcatgagccactgcgcccggcctgatttcctgatttcaaagatgtttttcccagtccattgtgaagcacaacccaagaaggtcacctgtctgttgttgctcttccactgcacagctgagagagaatgaagctgacagacactcagctgggaaggcctggcctccaaatcggctcctggtaactggaggggagctggagggccgaattcctgcagcggtcaccgccctgaggctctctctacagcctctgcacaccgagaacccaaaaagaaaaaataagtaaccaaaccaaagaaaatggaacctagttagtgcctcaatgcccctggacttcagtgctgatgtagtagatgataaagttgacttgatgtctgagatgctgctgcccctgcccagaccttctcctctaataacaaggattttctgagggaaatcacatcagggcattcggggatggttccccaaatgccctgcgtggcagttatctgactgtattcaaatttaattttgttcctcatatgaatcccatgaacaaatgattttcatttggcttatgctatgcaacacacagatgtgcatgacacacacgacagaaacacgtgttcacacatgtaatgcaggcacacacatggatttgaattaagcacagcctctagtggagtatctattttttaaggtagtgaaacagacttcatatggaacagaatagattaaattttcagggaaatttaaaaatacaaatatatgcattatttcacaatggcatgttgtttagggaagtctagccccaaaatgtgtggcaactgaaatggaatctggtgtttatggaatggaccacgcaggtgacagatatcctcacatcctagtacaggatctgctttcactaagtgtatgaacaaacagaaggataaggcaggaagcccctagaatactttccagtgcgtgtcccagggctcctctaggtgagcggagggctccaagctccccaccgtgtctgtctggggctgtgctcatgggcacttggccctgcgcaggaggaatgtctatgtgcaggaagcagctgccctggctggggctctgccccctgctgctggcccccagcccaccctgtctgcctccagagacccctctgccttcacagccctgggagccctgcatccagcagcccatgcccgtgtcctctcccaaggccggggcctgtccttcagctccctgctgtcagttcacacagaatcacagacactgcagcttacagacaaaccccgtgtggcattcattccccaacggcagggcctgaccacactcagatcacccaaatccatctgtgaaaaaccacaactatgagaagagccttccttctgctgagcccactgagccttcctcaaagtctaccctgggctccatcctggcctgccctccatgcagggggagcagtcctcaggccctgcccctgctcctgatgcccccacccaggggggctccttggctccagcccctccccccaggctcagtccagctgggatgctggtctcagcccacccagctctgcttgacttggtgggtgcagtgagggccgggactgagaaaggttgaagcaactccatttcccctactgcccatttttgccaactacggacacctgcctgcagcatctcctgcctggtgccaaagagcatggaatgatttgtgcactgatggttatttggggtatgtgagttcctcgaataagacccctctcttggacacccccaagctcaatttgaaggcctaagccacccagttcgaccttctcacacccaggcaagcctagcatggggcccccaggcctgaacaggtgtcctgttcagagggctcttctaccaggatggtaccagcattgtggaaggtgaatggggacagccttcagagtgccaccatttccttaaaatggcctatcacaggtaagccttgatatgttatcctttagactctgcaccaaaccaacaaactgcagcataccaccgttggtcagtgtgaggccagtactgaggctcatcaattggaacggatcttggatggagtgggtgcctttgcctccttccttcctcatccaagcaagggtgtggtgacaatgacctgatcggggtttaacgccggctctgtctgctcaccagacctggggtgctgagctctgaccagcctgggcagcccaacccacaggaactgcggtttcatagctgggtcttcaggaaggggtggaggctttgggagtggcagctccccgcctcccaccaccccaagccagagaatggggcaaacttgtatgcatggcttatctctaaattactaatctgcttcggaccagactcatctctacagtatagagttagagttattgcttctatgacaggtgttccagaagccctggtggctttaaagtctgagaaacacgggctggcaacttgggttgctgggtctgtaggggcgtcctcctgcaggatacagacaccccgcaggcatggaccacccgggccggcatggtcccttgcaagcaactggaagcattccggggctgtgttctactctacggcatcaggcatgaaaggcatgcaagggtcgcgaggggagcacacagggtcatttccaaagggccacagcatggccaagcaagggctgaggtgggtgtggggcttgtcttcatttttggtacgagtaaacaggcagcacctgtcactggtgcactatttacaaagcctcttcaataaataatttagagagaatcctacccgaatggctctaacatttgtacatgaatattgtacatgattaaaaataaataaggcaatataatacagttttcccacaaataaaaaggaagttgtttttcaccaaaccccaagggacattatggctaaacacagttcctgaactcccaggaagtggctggggtttggagttgctgatgatggagatgtttgcccctgaagtggagaccttgccaagtctgccatggggtcctttccagaacagtcgtgagcccagagaaggcagcatggtccccgcgacggcttcctctcactgccctacaagtggccacaccttgggcagcttccaggatgtacatgtgtgacctcccggctctgtggaccccaggcacagcatggcgtggctggctctcttctcagtctcacaggccaaaccaaggtgtcgctggactgggctccactcacgcctggaggctctggggcgaatctgcttcaggctcacttgggttgttgccaaactcagctccttctggttgtgtgagcgacacccggcttccttgctgactggcgctggggttgtggagtggcctctggtgttggctcctggccccttgtctttaagccagcaatgacggcaccatctctgtgacacttcgaatctttccaggctctcctgcctccctcagccattccaaggggtcactgagcccacccagataaaccaagttcccctcccatccttagatccctaaccctaattccacctgcaaagtcccctttgctgtgtgacagcacctggccacagggcttagaactggggcatggacacctttggggttcactcctctgtctacccaccacctggatggccgaagctgggcagcggcactgggggcaacagggttggctgtgccaggggctctgcacccttctcaacagctcgtgggtcaaggacagcaccacggtgagctgggggagccagggcagccacactcaccaccaccgcactactccctcacaggctccctgtggctcctgtctgaagtgactgctttaaatccggctgggatagacagatgaggatgagaaaatcctagtggaaaggggaccataaggacaaaccatttgtcctgaagagaggaaagcacaggagcagggacaaggcagggcctggaggagaggttgacagcagggccccagccaggatctcagcccacagccagctcagatggaccctgggtcctcaggatgagctcaggagccctcgatggcagcctggagattccacataaacattaggtcctgtggatgtcccagtagcagcgagaggccctgcaagcacctccttctgccctaggacctcacgggagcccagcccccaccggcacaaggtgatgccagaacaccaggaacatgagcggacagcgacatgaggaccacccaaggaagatgaaaggtgcccgagctctgccctcaaagtctccagtgggtccatggggtcagcctacctgtggggtcatgtggcctggcctgggagctccctgtcataaccaggggaaggtgctggaaaggcattggtcaaaatcactctgcaagaaggtgtctggagaccatcctgcctcttgcaccatcacagaagccagagcctaatccacaccctaaggacaggcagacaggggcccccacatgcagcctctacccgccttccctgcccgaagccatccaccctgcccacctctgtccggactcctgtctcagctggaagcgccaggcatcactgcactggccgccctgcaaagccctcagggtctggcctcccccagctatggcccaggcccctgctgcccccacatggccacacagctgaggcaggatcagcccctccctgtgcagggggctgcctctgacggcagcagccaaggacatcacccacctgtgcggacagggatcagcctggagcaggtcccacacacaggtctacactccagggaaggaagtctgggcttctctctgctcctattctgaaaagtcggggccctcaggaaagggttacagctgttgaggagcagtgaggaggcggacccccaaccctgctggctttgagcataggcagggctcaggcctcatctgcagtccacagaaacctctctgaccacatctcagagcagtgggtctttagacattcccctactatggtgcctacccagaagcttccctcccatttctagctgccttcctccctgtgaccgagatccaaggtttccacatgccagacctctgtccactatttctggatagtgccttcccagtggccctcctggaccccgtccccatcatccttattttcatcttcattgtgactatttagacatgcacataggaggttgtcagacgtcagacgtcaacactatcacctgcagtcaatttccctgcaaattacaacagggacacctgcactcacgaccatcagccaattctgaaacttcgtcctggagggttggttctgccggagaaacagcatcttccatcaaggaaacttgctcatgggtgtgacagccgctcatattcaacagaagtggagcctcacactgttgttgctaaatgtaaaggatccacgatgccacagggaaaagaagaaatgacacccttcgttttctctgaacaaacacagtgccggtgcaggatggggaatgtccaggtgttttaggagctggaagccattggcggaggggtggagaatgcacaggtgcagcaagaagccgatgctggccatggttgtggagagggggtcacagggcccccctgagaactccagaagacctgcctctggctcttagcaaaaaaccacgcttgaaagccagcagccaccactatccatgcagtgagaggcagcttctcaattctccccagacggtccagttcaagagtggacagctctgtattgtgcctgtggtgtgaacaaccccaggccttgtgaccttcccagagaggcctgacttcccactctggctcttgaagccgctgcccagggctggagccgcctgtatgtcaggtcccacctgggcggggcggacagggctgtctcagagggcacactctcgcagagctcctcagttgctctgccagccacacctcagtggctcttgctgtaaccctgggatgctctgaaggtccttacattgatgccgacctggccaaacctgaacaggcttgctggaaagaaacagtgctccctacgccacggagggaaggatggagtggacacctctccagggaggcctggaagtgtgcacagtcgggtgtcctcccctcaccgagtcactgctgtgctgtgcctgctcggtggttggccctcgggccacaggccatgcctggacaatgctcctcctccaccctggcaagtggctccctgctctgctggtctggctggtcctggctggagccaccgtggcctgtgtcacccccggagcattcccaccccatgtgcaccccagaggcccacgtgggctccactaagcctccttcccagctgctgcagagggcaggtactggcctggggagtgtggagggagcccagccctgactgagacgccaggcatggggcacacggggggacgtctgccctgaaggccagctctcccaaatggacacattttccgatccaagcccagggacctgatttgggagccgtttccatcagtcctgccttctagaaagtatgtcaacatctcgcctttgcccttgacactgactttgcctcggcacacaaagtggtaggggcaccttctcagcagccggtggacttcctcagtcacctggattctgccctggacccctgtgctatccatccgactggccacgttgactgtgtttccccagatgtcgtactggggcctgcgagcgccaatcactccagccaccacagggccaacattgatgccaactcggaggacaaagtcgttgtaagactggtagttgatttcatccagaacgtcaaacatctcaatggcaaagtccgccagcgtgctcaggtgggaggagatggacttcttagccttggtccccgaggtgggcgctagccccacagcggccatgtaggtgctcccgatggtcttgatcttctctatgtccttgtaaaagtctttttccatgagctcgtcaaagtcggcgatgatctcgttgagaagccgcagacactccacccccatgttgttgccgtccagctcgatgtagaagtcattgaagttggggatggaggcaaacatgacgcccacctgggagtaggactggtagtagaggtccatgttccgagggttggacatgaggaagtgctgggcgacgtgggccggcaggaggttgaagaggatgcgcctgttgtccagcttcaccttctccatgtcctctcgctcctcctctgcctgtgcggcccagaggtagtccagcctcagcctgatgtccacctgcctggcatgcagggccagcgcacaggagaagagcaggatggccacaatcggctcgtagctgcgcccggagacggcaccacccccagtcctggtgtatccgctgagctccagaacgaggatgtaggacgtggtgagcccggagagcaggatcatttttggcaaggaggacacccggaaaaatatggctagcgggagggtgcccaccaggcagcagagcagggcatggtgtgtagactcgcagggcagggtgggcagggctgtgcgctggcccccagacgaaaggaccaccagggaactgttgggcttggagctccaggcccaaggcaggcagcccaccacacaaccttgggctactgagtagattaagaccactatgaaaatacacaggacagtgcgaatctgaatcgtcaggcaccctggaaaacactggacccgggtgatgtgcaggtacaggacacaggccaccaggaagcagatgcagaatactagcaggagcaggacgaccacactctgtgggaatattagaaggtagacaaggccaaataaggcagccaggatgagggtgaggacaacggcgctggtgaaatactcgtcctgaagctggtggtacttttgctcccgttcgacatgtttgtacttcagggtaaagaagttcaggtctgccatctccagctctgtctggcgggcttctaagaggcggctgatgtacctgttgacgcgagtgcccggggtggtgtagacaacgttggtagaaaaagatgagcggtttctgagtttttccgaggctgttcttaatgccctccgcttgtcatcgtcctcgcaggtcatgacattggagaaggggatctcggccttgaacattttccggcagtgcatgagctgcaccagcaggtagcagacagtcttgaacttcatccttttggccggttttatatctgagagaatcaggcctggaaatatctttcggcgatgggatggcacaataaaaaaggtttcgatgttatgagttttcaagaaactgttcctctcatgtccgtaacccggttctacctcgtagtccccattcaagcacgctagggtcgtctttgtgatatgaaccttccctggcaggccagcggcttccatgacattggccaaggtcacatcattggaccacacgtcgtactgccacttgcgcaagcccaggacaccacagaggaccctgcccgtgtgcagacccacacgcatgttcagatccacctcggtggcttcagccacagatgtgatggtatcaatcatgtcgagtcccatctccacacagcagtgggcatggtcagtcttgggctgggtgaggcccgacacgcagtagtagcagtccccgagaatcttgatgcggcgacagtggttctccgtggctaattcatcgaacttgccgaagagctcattgaggagtttcaccagctcctgggctgtgcactgggatgccaagcccgtgaaacccacgatgtcagcaaacaggatgctcacattgtcgtgcctctggatgtaaatcttgtggaaaatcctctcagggggcttcaggaagtcctccttcatctccatggcaacgttccggggcaggaggctcatgaggagccgctcctgcttctcgttctcatcctccagcctcagtcggtcctcaatgcagctccgggcctgcaggaacgccttcctctgtgaacgctcagtcagaatccgcacaaagaccccatacatgttcacaccgacgaagagcaaggcattggcaccgagcgtcctccagagacgtgggcgcttggcggggaccaaggtggctgtgaccagcaagtgcgacgcagccaccacgagcccaaagcctatggccagcaggctgcgcacgggcagcaaggcataggacacgaaggtgaccaaaaggagctgccaaaccccttgttcggcggtcgctggccccccagcggccccggcggaaccccgggcggggccgcccagcgcgaaaggacagcagagcagcgcgaaggtgaggctgaagagcagcgccagctggccgacctgctgcagctggggcacctgcagggaccggacgttggttaccacgagcagcgccaggaagaggacgcagtgcaccgggtgtgagcccttggccaggccgggcgcgggccccggcgcgcccagcagctcggccagcgccagcgcgcccgccagcaggctgagaacggccagcgccttcagcgtggccgcctgctccagccgcagcgtgtagccgcggaacagcgcctccagctctgggcaagcgaactcctcgtcgcacgcccggagcccgcgccggcggcttgtcccggccgcccgctcggcgcccccgggctcgcccgcgccgcctccgccgccgcctccgccgcgcggcgcccccgccatctcagcgccatgcagcggccgcggccgcgggcgcgcccctcgccggcccggggcgccggggcgcgggcggcggcgccggggcgggcgggcggcgggcggcgaggcgccggggcgcggggcgcggggcgggcggagttggggcgccggctgccccgcgcgcgcgcccggagcgcgtc

SEQ ID NO: 15343 - RNA, 1639 nt, Homo sapiens
  source 1..1639: mol_type = other RNA
gctgggattacaggcatgagccactgcgcccggcctgcactgtgggttttaaaacacgcatagagtgtggcagccatggtgcccaggccatgcagagagacatggggacgtgggaaggttcttgtatcaccgtggagtggtgggtttcacctgcaggagccgggggtccacggggacgtgcactgtagaccccagagcagccgtggcaccgacgtccttgcgggttgttcagagacgccagagtgtggggggattcagtgacttggggtctcatgggctcgttggctgatttctgtctggagcacgcgccggctctctcccattttctactccgttgagaccaaattaaaatggaaccggccacaaagcaagtggggcttcgtgtccacttctccgaggctggggccgggggcatcgccttcctgggagtgcagaggaacgcgggcagagtgtgtgccatggccttggccagaggcgatggagccaacgcaggaggctgcacctgccttccccgaagtccaccgacacctgctgtgaccggacgcatggcaggagcagggagggcgtgggaaccagggtgcctccactggcctctggcagagccggagctgctgacgccaggacccgtggcactgaacctggacacatggctgaatgccagggcccatggcactggactcagacggatggctgagtggggagggattggtagaggccagtgcccagctcttcccatctgaagacaggcagaggagccacggcaagctcgagctctggaggctggaacaggtgcaaggctgggtccatctctgttctccatggacctaggaggagatgtcgcggttcctgaatctgaaatggacataacaacattcctgctctgaggagctcccgggaagagcacataagccgaccgaagcccctgtgcctggcgccgaacgtgctctcaacccacacccggctcctgacacgccctcaacccactcgctggcagggtcaagccacccccgagtctgcctcagcagagtccccaaacctgaagctggcagatttgaggctaaaaaactaaagacagagctccaggccggaggccaactgtccttccccaggaacgagaagaggtctgtggtccggatgagcagaacaagggccggaggccccttgcagggagcggagcggacagaggttctgttggagccgcagctcagagcccctgagggaccccctactctggggccctggcccttaccacagagccttgtgtgtgttaggaccgcctgcccaagaccggcagagccagggaatctgcatgtttaacatggcctcagattccacgtggggtgggttatggtgggggagaccagagaggaatccttgcttcacagttcgaagtcggaagacaacgttagtgctacacagccggggagcagcaagccctgcttgtcatgcagagacccggggctgcgtttcgggaatcaggggagagaagtctaaacggggctgtctccagggagaacgatggatgagaaggtggggccgctcttgtttgtagcagccttgtaaaactggcatttttgtttttgagacagagtctcgctctgttgcccaggctggagtgcagtggtgtaatctcagctca

SEQ ID NO: 15344 - RNA, 2030 nt, Homo sapiens
  source 1..2030: mol_type = other RNA
gctgggattacaggcatgagccactgcgcccggcctgcttcctgccaagttaaacggcatgctagctctcagctccccatgcccaagtggacttgaaaggtctaccccagccctccttccacagcccatcctgagcaggctgcctactccaggcaggccccaggctgggctggaccatttaatcctcacagccctggtaaggctgagatcacggatcccacttcatagtggagaaactgaggctcagggggtgctgaatctctagctctaggtgtctttgctctcagaagttggtcggggagggggtctgcttgctctctgggcacgtgtcctactccctcccgaggggcactggagcaaatcccaggtccttagccagcaaggagaccgctgaggctcacacctggtgccgcccacccagaactggagactgagatgctgactcacccaggagtggggaccaggagggccccgatgcagcccgaccctcctctgtcccagcatcatctcgcctggggtcgcgaagaccccgtgttccctcaaggcctcagaacaaaagcggtatgagagggtctgggggtcctgctcccctgctccaattctgggtcccctggctggtgggcaggaccaagatgtccctaaggactgtccgggcagagccagccagggtggggtgagggctgaagggacagtggctgagggtctccttggaccctcccagctgtggtgagtggccggagggggaagatcaaggccatcccagctcctctgagctgaggctgactcaggctgtcgcacacctcatgatcagctcccagtcaggtggtccaccctgagtgtccctgcgtctgcccccatctgcacccccgggaggtgccttgggggaggctgtggggtgggttgcaccctaagcacgcactctgggctcctgacttaatctctgagacccccaccccctcaggctggactggccacctgggctggctgggtcccctcacacctactgggttctgactcatggtcccagcaggctaaaaagggggtggggcaggacagcccagtgggcggagctgtgagaatccaggccggcctctgggctatgctctgggcaggtctcatgccctcgtgagccgtggtctccccactgaggcaaggggtcagctgccagggcccccgtcatcagccatcggagctggagtgcaggtggggaccaccatactgattccaatggccccagcctggcccccacaggtcccccaggccaggacttcagcctcctagagcctacagtgctcaccatggggggacccagcccacaggtcgggctctataacgtgtggcagagacagaatgggagacaggcccctagtccaccctggtcgtcaccacaagtgccctccccctgggcccccagccccacctgggagaagcagatgtgactcagtttccctcattcggcctttctcgttctgggctagacttacccaggtggcatcttgagtcatcctgggcgatggcaggtggcctcggggcatgagggctgcactccaggatgcccggtggctaggtgacaggagaggccagcgcaggagcttctgtccccagggagtgctcgaggcaggctgggccctccagagccaggatggcaggaggcccagctcactgtgaggaaggccagccccaggcaggggctccaggtcagcgccacttcttgacctgagggtggacacagtcccttgagcttcaggcatcacctggggaggtggccaagggtggaagacctgggccgttaggtcccggaggatcttccctagcccacgatgggctcctgatgtctcgggtggtgctctgggacggggccacatttatctcaagctgaaggcgccgtctccacgccgcccaggcttccaaatgcggccacacggactttgaagggcgtccgctgcagggtcacaggcgccagtgtctgctcgtctggacctcgaagcaccaggcccaggaggagtcctcctctcatcgagttgaaagaa

SEQ ID NO: 15345 - RNA, 2181 nt, Homo sapiens
  source 1..2181: mol_type = other RNA
gctgggattacaggcatgagccactgcgcccggcctgcttcctgccaagttaaacggcatgctagctctcagctccccatgcccaagtggacttgaaaggtctaccccagccctccttccacagcccatcctgagcaggctgcctactccaggcaggccccaggctgggctggaccatttaatcctcacagccctggtaaggctgagatcacggatcccacttcatagtggagaaactgaggctcagggggtgctgaatctctagctctaggtgtctttgctctcagaagttggtcggggagggggtctgcttgctctctgggcacgtgtcctactccctcccgaggggcactggagcaaatcccaggtccttagccagcaaggagaccgctgaggctcacacctggtgccgcccacccagaactggagactgagatgctgactcacccaggagtggggaccaggagggccccgatgcagcccgaccctcctctgtcccagcatcatctcgcctggggtcgcgaagaccccgtgttccctcaaggcctcagaacaaaagcggtatgagagggtctgggggtcctgctcccctgctccaattctgggtcccctggctggtgggcaggaccaagatgtccctaaggactgtccgggcagagccagccagggtggggtgagggctgaagggacagtggctgagggtctccttggaccctcccagctgtggtgagtggccggagggggaagatcaaggccatcccagctcctctgagctgaggctgactcaggctgtcgcacacctcatgatcagctcccagtcaggtggtccaccctgagtgtccctgcgtctgcccccatctgcacccccgggaggtgccttgggggaggctgtggggtgggttgcaccctaagcacgcactctgggctcctgacttaatctctgagacccccaccccctcaggctggactggccacctgggctggctgggtcccctcacacctactgggttctgactcatggtcccagcaggctaaaaagggggtggggcaggacagcccagtgggcggagctgtgagaatccaggccggcctctgggctatgctctgggcaggtctcatgccctcgtgagccgtggtctccccactgaggcaaggggtcagctgccagggcccccgtcatcagccatcggagctggagtgcaggtggggaccaccatactgattccaatggccccagcctggcccccacaggtcccccaggccaggacttcagcctcctagagcctacagtgctcaccatggggggacccagcccacaggtcgggctctataacgtgtggcagagacagaatgggagacaggcccctagtccaccctggtcgtcaccacaagtgccctccccctgggcccccagccccacctgggagaagcagatgtgactcagtttccctcattcggcctttctcgttctgggctagacttacccaggtggcatcttgagtcatcctgggcgatggcaggtggcctcggggcatgagggctgcactccaggatgcccggtggctaggtgacaggagaggccagcgcaggagcttctgtccccagggagtgctcgaggcaggctgggccctgcagacaggcggtgcacacaacagagcccagggccagagagtgagtcttcagggtgtggaggtgaggctgagcctcttccactcagacgccctccagagccaggatggcaggaggcccagctcactgtgaggaaggccagccccaggcaggggctccaggtcagcgccacttcttgacctgaggactcagcccaggcctctgatggggaccgccgatccagagccacgggcagggcctgagggtggacacagtcccttgagcttcaggcatcacctggggaggtggccaagggtggaagacctgggccgttaggtcccggaggatcttccctagcccacgatgggctcctgatgtctcgggtggtgctctgggacggggccacatttatctcaagctgaaggcgccgtctccacgccgcccaggcttccaaatgcggccacacggactttgaagggcgtccgctgcagggtcacaggcgccagtgtctgctcgtctggacctcgaagcaccaggcccaggaggagtcctcctctcatcgagttgaaagaa

SEQ ID NO: 15346 - RNA, 5126 nt, Homo sapiens
  source 1..5126: mol_type = other RNA
gctgggattacaggcatgagccactgcgcccggccttcagcttaatttttaaagcactttttggttactgaaatgatattatttattgtttatctctccagtgtgtttcaggagagcaggcccttgtccgtctatttgccaccacatcccctggccgagattgggtctagaacaggttggcactcaataaatatttcttgaatactgggaaaacaacacaccagaaatggagcattccttgacgctgcgcttgcttctgagtctccacgttgctttttgtgcgaatctctgagtctgtctccggcttacctctccctctctatctctgtctctgtgtgtgtttctgctatctctgggacttctctgatttgtgcacctgtcagtctctcctcttcctcttctctctcctctgtatcaccttcctgtctttgactttttctctgtctgtgactctactagtttggtctctcctgctctccccctccctccccatcttgctcttcctcctgcctaccctcaacctcattctttctctctctctctctctctctctcgttctgtttggccttcagactctagaatccattctcccctaaccagttccctctccctcttccagcaaatatttgctgtctctcaattttttttttttttttgagacagagtctcgctctttcgcccaggctggagcgcagtggtgccatcacgggtcactgcagcctcaccctcccaggcccaagcgagatcctttcacctcagcctcctgagtagccgggactacaggcgtgcaccaccacacccggctaatttttgtatttttggtagagacaagatttcaatatgttggctggtctggaactcctgagctcaatctgcctgcctcagtctcccaaagtgctgggattaggagccacagcacccggccagatttgtctcttttaacacccgctccggcatccctcttctctccacgtatccgtctctctcactcagcgcttctccgtctcactgatttgtattccttttcctacatttcccagcatctcttcctgaaaccgccttggcagaattcttcctagggaccttcagtctctctcttcctggtccttccacacaggcctcggagagaaattctgaacacccagctctgatctgtacccttccgtcaagagaagggcacgcagagcccctggcagcatggcaccaccgctgccacgtcctcctcaagctgcgtctgtgcctgttttcccgccagactgggagccccttgagagcagggcaagatcaaaatcacctctccactcccagcaccgcccagcacaaggcttcgggggaggcctcaggaaacacttgctgagcaaatatggaagggaagcctactgggcgctgtcccctctgccttctcagtgaacttcaaacccatcccctccaatcaccgcacagcccttgcccccgcgcagctgtcatcctctctcaccatccttagaagagcctcagtccctctgcctggaactcaggcacctttttctctttttttctgagacaggatctcagtctgttgctcaggctggagtgtagtgccgcgatcctagctcactgcagcctcgaactcttggagtcaaatggtcctcctccctcagcctcctgagtagctgtgtccacaggtgtgctccaccacgcccggctaattttttttaatgttttgtagagacagggtttcgccatgttatccaggctggtctcaaactcctgggctcaagtgatactccagcctcagcctcccaaagcgctgggattacaggcatgagccaccgcgcccggccaccctggtacctttacactctagcttgtggctactttcccggcctcatctcccagccccaccttgtacatcagcatcccagaactgttagcactgaccccaatacatcatgctcgttcacttcctcccgttttcacccaagttgttctttggccccacaagcctttctcatgcctttcatcaaccagaagatgcccactcatttcttcaagacccagaatgggcatcatattctccaggaagcctaccccaagtgctgctcactcctggcagttggtcactctgtccaccgtgtgccacggtacccacggtggtccgggttccagcaccgattgccctgcctggatggcggtgtttgatgacaataaactgcttgagagcagggctagagtctgtttcacccctggggatctggatcctaacacacttcctggtaccttagcagatggccaaaaatggcaatgggtgagtggctgaatgaacgagtgacagacacatgagtctctaagccccacggctttctcctgcacaccagacaccatgactatgcttcagcatctgtgtaattacgtgcttcctcccacaagagtgtgagctccaagggcccgtgcccatgtttgatgctgtatttcagcacatctctgcctcctactcttgcctccgagttcctgtcttccctttgtacaccattcacgttagcgtcctgcttaaacccgttccacggccctcaccactcctagaataaaatctgaactcctgacctacgagcccctgcacaatctggccctgtctgtgtctccggcctcaccttgatccccgctcacctgcctcactacccttcagccctcgctgcaagctccttcctgccccggggcctttgcacgtgctgctctgcctgccacactcctgccccagctccgccctgctggcttcttctcatcctttcactgtccactgaaatctcttcctcacaactgggttaggctcccctgatggagcatttcatagcatctcgtttctcctatagcctaactgtaatttattgtgtatgtacatgatcgattaatgcctgtctcatgcacaagatgtttactctatgagacgtcggggcccctggctgttttcctgcctcctgcacgctgagcacggagcacaatgcctagctttttaaggcgcacaaataaattgccggtaatgaatgaatgaatgagaaggccctttctgtgcctcgttcgtgtcccctgctccaatgccttcttatgtaccagtgcctggtacacagtaggtgcttaataagcccttgtggaataatgaatgaaaaaaatgaatgaatgcccgcgtccaacccttctttctgcctttctgcatcccttcgctgtgtctctttatatagggcatatatatagtttgtgggtgtaactatgtattcgtgtattatgggcccctctccaggagttgggctgggctgggagtccctccctcccctccccccgccccgccccccatgcacacagcaaaacatgaaaaagaaaacatctcgaaactgcaaaaaacaccatggccctcccccctccccatagatcccccaaaaaaataaaacacgacgctccctcacagcggccccctccctcccctgccccctccctcggggtccctgcttcggagggggaggggggcggggagggtgggcgtggggcgggcccagcagtctccagcgcgctcacgggggaaagcgggggcgcccccgaccccggcagcctcgatgcacgcgcgcccgcgcacgcgccccggacacgcccctcggctcccccgccgcgcccctacacaggcgtggttttcctgttgagcgtgttggtgttggaggcggcggcctccttggccagggtcccgggggcgggcgcagagggcgcgggtggcgcgggcgcgggcggggcgggcggcccggtgaccgtgaccgtgacgccgccgcccgcctccttggggaaggcgttgtgcagcgtgaggaagccggacgcccccccgcggtcccgctcggcacccgccccgccgccgcctccgccgccgcccccggcgcccccggccgcgccgccgaacgcccccacggcgccgccgccgccgccgccggcccccgccagccccgcggccacgctgcccttggaggggtcgcggctgagcgtgtacatggagatgtccgtggaggcaaagcccgggcccccggggccgccgggagacgcgtcccgcgacggcgacggctcgctggagcgggagctagagcgggagcggcggcggtagcggaagcggtaactgggcagacggaggatggccgaggggccgctcccgccactgccgcccgcgcccccgccggccttgagcaggtccgagcgagactggcagtgcgcctcgcggctgcgctcgatgtagatgttgacggccagcacgcctatcacctcggccaggatgaacgacagcccgccgaagtagaaggaccagccgtacgagtagtggtttttcttctcctcgtcccgcttcgggcccggctcgcccgcgttggcggagatgtacacgatcacgccgatgatgttgctcaggcctgctgccacgaacaggatccctgcgcccagaatgatgttcctcttggacttgtagacgcgggaggccgccacgcacacacccccgagcagcagcaggatggcgctaaggatggggaagatgctggaggcccggacaactcggagtagatactccgcgctgtcgtggtcgtagtccgtgtcctccgggaaatgattgatcttcacgcagacgcctcttttcaacccttccaggcagcagatcctccagaggcccgagtgcgtgaggccgccggggtccttcttctccgaggcgccgccgcccccgcggtggggggtcccgtcgtcgccgccggccgtgaggttggtggtgttgcagatgagggcgcgcgtgtagagccagtagtcagtgctgatggcgatggtcatgaggccgaaggcggcgaaggcgcccaccgtcgtcagcagcacctgcacccccttctcgcaccagaggccccgctcttcgttccagcgcttcagcgactccagtttgaccacgggcagccggggggccgtgggccaccaccggggcagcgggggcggggccgtgccggcggctgggggggggttcacagcgcaggcagaagcggggggcccggggccggcggggctggggaggggggcggcgaggaggaggctgcggccggggagggggtcagagcgcggccatggtcggcggctggtggagggcaagg

SEQ ID NO: 15347 - RNA, 943 nt, Homo sapiens
  source 1..943: mol_type = other RNA
gctgggattacaggcatgagccactgcgcccggccttgatgacgtctctctttcacttttgttcctgacagtccagactgcacaatttcggatgtgggagactgggtgatttctttgatcttcccaaccaaatatgacttacttaaggattttaccactaggtaaataggtgcttgactgtgatttaacacctgaattactaaaattgattgcaataattatccaaagaaaaacagccaagtgcaacagtaacgacagcctctgaactctctccacatcttcttgtggacagcctttgagctctctccatgtcttctctgggacagcctctgaactctctgcacgtcttcttgcagacagcctctgagctgtttccatgtcttctccgggacagtctctgagtctctgagctctttccacgtcttctccaggacagcctctgaactctctccacgtcttctctgggacagcctctgagctctctcttgtttgggacatcctctgagctctccacgtcttctctgggacagcctctgagctctttccacgtcttctccgggacagcctctgaactgtctccacgtctcctccaggacagcctctgagctccctccacatcttctctgggtctcctgtggagtctgatcacctttcagttaaggcatctcctgtgagcaacccagttggctactctgagttctgggggtagctgtccttggtttctctgaattgcccagaaaccaacctttctgttgcccatcgtagtgcctacgtggcttagctggagccctaccctgcttttgttgcccaaccaatgcctatgtgacagggctaaattcccattcagctttaactgcttagttttagaaaacaggatgtctggggtcagaagttccttcttaggactaaactggctgaagctggcaaaatccgcaatggcagc

SEQ ID NO: 15348 - RNA, 3880 nt, Homo sapiens
  source 1..3880: mol_type = other RNA
gctgggattacaggcatgagccactgcgcccggctgatttattttgttaaataagttaatgtgcagatctgaagttaggtaattatacacaggcattttcctgggacaaacttcaagtgccaggtacttgcactcttaatactgtcttaccatccagttataactggacaaaatatacacttgagacacggaaaaggtcttagccttaaacatgatgacattgtaagcttcttacagcagtgtaattgaggcatggagataatgtcttcaaggttccccttctgtgtacatgtcttatgtaggataatattcttaacattttattcacttcaagtcaccccattttgccctgatttcttctgaagaacagaaactttggttataagaagcacttctgggttctgacagacagtgaacctgctggagtcggtggtggggaggaatggtaggtaactgggaggtaaacaaacaacaggaacaataggcaaggttagaaattgaagtgggagaagttataaaaatttattttcccacgaaataattccacaagctgtgtaaacatttcttactaaaacaaatactctaacacacaaagattgtacatttccagtgaaacactcacagtaaaattgcctgtattttcactctctaggagcaaaaacaaggaggcagcagatgaatgctttcctagttacctttggcagcaagcttactcacattccctgactgctcaatgggttgttaaagcaacatatagcacaattaattaaatacagagcgaggtgggcagaatgctcgatatcagtctctagtttcttcgttagtcttcagcattccaattcatctcaaccattcagtcactcggtgcacactttcttacatacggacacacacacgtgcatatagcgagttccggctcgtagactccagtgcagtgactagaacagacactagctactaagaatgtgtcacaatcagtgtgaactgtatggagtagaacaacctctggagttttatatttaccataatttatggtggaaattacaaacttacttacaaggatggtataacattcagaattcaaaccttttcaagtcaagcaatcacacatatttacagtatgtacacactttctactagaatgaggataggtgtctagacaatgttattacaaatttcctgaatgtgggcatttctagtccctgtaattcataaagcaaatctgctgacttggcattaagactctaaaatagtgtgatcaaactgatatatatatatattatatatataataagaaggtgtttgtttgcagaaataacatttacaaactgtctatacagtacacagtactagtacatagaaaatagattctaactttatgatcccctttgtgtaaggcaagactgaatctgtccccaaatttagtcagccagaggtacaagcaagaaacagtggtccatgaatgaatatgcaaatcagatgcctgcgtattaacgtattaaaaatctggagaaacaagaaattccactttttatctgtgctgattctggcttgttggatacatcaactacatttcttaaaacactaacatcacctgggtggcaacagattttgttcaagtggcagctacccaaaacagtttttgaagagtccagtatgcaaccggaggactgcagccataccaggccaatttatgtagcacttacaaaagaaaaagtatctcaatactctatccatgctattgctattcaagcaacagcaataatacaaaatattacaagacagatcacatatgattgcagtgtagaccccaaagactttgttttggggatgctgttagttatacaagacttcaaaaaaaaaaaaaaaaaaacacaaacgggcaaaactcattggcggatgtaaacatccctgttccactccccagcctcattccgtttttttgatatcacttctccatccttttcacagtagcgatccttggatttatgacggctgcgctgcttgttgcactcgttgtggtcctgctctcgatccacgtcccgggaacggtgccgggactccctgtgtctgtggtcactgctcccgtgggtctcgtctctgtggttgtggtcacggtgtgaggcatagtggtccacgtggtcatgggaataatcttcctttggctctacgtaggcagagtctcgactctcctgggtttccgagtcaaatgtctcttgcctggagaggccgcgacttgtcccactgcgatggttgtggtgtggggctgaggaggaagagcggtgctgggatttcttgactggttccacactaggttcttcttcagcttgggaagcagaacggataggagcggagcgatcagtcctctgatcaccttgagaaccctgtgaattagaggctagggtggggctaagaggcagacttgaagtggctaatgtacggctaaggagagggttggggaggctactgctgggaggatgggtggccttccagtaggcctccagatagtcggcaaggtgctcacaggcatcctcaagctggttctcatccaagatcacatcgaacagctctggaggacactgagccagtttatcagctgctaccatctggacgttgaggtgtttagcttgagatttccctcgagattttattaacctttgtaaaaccttaggagaagaaatctttacatatactataataggggccaaggaggttttactgagttgagctggatgattaattgtatccgcgtcaaggaccaccaactgcaatgttcttgcaagttcaaaaatcctttcgatttcactctgaacttccgctaagcttgaccttgtgttggatctttctattattgcgtgcttactgggattgtttaataccgagcgtttggcaagcgagatgtcagcggtgacccttgtgatggatatccgcccttcaaatctgtgttttaaaaaatcaaacagcgctttttgcatcatatctgtgacctcgtagcccttcagagaagggcccactaggaccactggtcgcatggaaggtaccacatcatacggaggagtgtgctctgtagtaaaccgccaaaacaagcctgcagttttccactggtcttgttcatctgcagattttgcaccagatgatggaggtgttgattttctggaactaggtactatgtcacccaaactggatgatgaatttcctcctgatttactggagtagaatttcccttgcttggctctctgttcatgctgcagcctcatgttttctagtttgactgggcttggaatgaatccgatttcacagccttcttttaccaatcgccctatccaccagtcattgttaaatttttccttaacatgcagaaaatcttttgcttcgaatgagatggccatgccaggcactggaacatcatcttcatgggccgcactgtagctgacatttgtccgaaccgcaaatgcaacgggctttgtctttgctttttccaactgtgcctgggcctgccgctccgcttctctgcgcactgcctcccggtcctcctccagagatacatcggaatcggatggacggctagtgtaggagtctgccgaacccccaggaataatgtatttagtttgaggagctataaggcgtctgtcaagcatgctagaccaattccaagtgcgcccagcactccagcaggaattttcttcacaggagcaagaattcaggactagctaaaaggcagccaagtcttgctttgctgaacagcatagcaactgctttcctttttcttgctggcttggggtgtgtagtcttagttagtgtgactttctaaagttcgtcggatcacaacagctctctgttccagaaccacttaggcagagcagaggagctcatcaaagtc

SEQ ID NO: 15349 - RNA, 4113 nt, Homo sapiens
  source 1..4113: mol_type = other RNA
gctgggattacaggcatgagccactgcgcccggctgatttattttgttaaataagttaatgtgcagatctgaagttaggtaattatacacaggcattttcctgggacaaacttcaagtgccaggtacttgcactcttaatactgtcttaccatccagttataactggacaaaatatacacttgagacacggaaaaggtcttagccttaaacatgatgacattgtaagcttcttacagcagtgtaattgaggcatggagataatgtcttcaaggttccccttctgtgtacatgtcttatgtaggataatattcttaacattttattcacttcaagtcaccccattttgccctgatttcttctgaagaacagaaactttggttataagaagcacttctgggttctgacagacagtgaacctgctggagtcggtggtggggaggaatggtaggtaactgggaggtaaacaaacaacaggaacaataggcaaggttagaaattgaagtgggagaagttataaaaatttattttcccacgaaataattccacaagctgtgtaaacatttcttactaaaacaaatactctaacacacaaagattgtacatttccagtgaaacactcacagtaaaattgcctgtattttcactctctaggagcaaaaacaaggaggcagcagatgaatgctttcctagttacctttggcagcaagcttactcacattccctgactgctcaatgggttgttaaagcaacatatagcacaattaattaaatacagagcgaggtgggcagaatgctcgatatcagtctctagtttcttcgttagtcttcagcattccaattcatctcaaccattcagtcactcggtgcacactttcttacatacggacacacacacgtgcatatagcgagttccggctcgtagactccagtgcagtgactagaacagacactagctactaagaatgtgtcacaatcagtgtgaactgtatggagtagaacaacctctggagttttatatttaccataatttatggtggaaattacaaacttacttacaaggatggtataacattcagaattcaaaccttttcaagtcaagcaatcacacatatttacagtatgtacacactttctactagaatgaggataggtgtctagacaatgttattacaaatttcctgaatgtgggcatttctagtccctgtaattcataaagcaaatctgctgacttggcattaagactctaaaatagtgtgatcaaactgatatatatatatattatatatataataagaaggtgtttgtttgcagaaataacatttacaaactgtctatacagtacacagtactagtacatagaaaatagattctaactttatgatcccctttgtgtaaggcaagactgaatctgtccccaaatttagtcagccagaggtacaagcaagaaacagtggtccatgaatgaatatgcaaatcagatgcctgcgtattaacgtattaaaaatctggagaaacaagaaattccactttttatctgtgctgattctggcttgttggatacatcaactacatttcttaaaacactaacatcacctgggtggcaacagattttgttcaagtggcagctacccaaaacagtttttgaagagtccagtatgcaaccggaggactgcagccataccaggccaatttatgtagcacttacaaaagaaaaagtatctcaatactctatccatgctattgctattcaagcaacagcaataatacaaaatattacaagacagatcacatatgattgcagtgtagaccccaaagactttgttttggggatgctgttagttatacaagacttcaaaaaaaaaaaaaaaaaaacacaaacgggcaaaactcattggcggatgtaaacatccctgttccactccccagcctcattccgtttttttgatatcacttctccatccttttcacagtagcgatccttggatttatgacggctgcgctgcttgttgcactcgttgtggtcctgctctcgatccacgtcccgggaacggtgccgggactccctgtgtctgtggtcactgctcccgtgggtctcgtctctgtggttgtggtcacggtgtgaggcatagtggtccacgtggtcatgggaataatcttcctttggctctacgtaggcagagtctcgactctcctgggtttccgagtcaaatgtctcttgcctggagaggccgcgacttgtcccactgcgatggttgtggtgtggggctgaggaggaagagcggtgctgggatttcttgactggttccacactaggttcttcttcagcttgggaagcagaacggataggagcggagcgatcagtcctctgatcaccttgagaaccctgtgaattagaggctagggtggggctaagaggcagacttgaagtggctaatgtacggctaaggagagggttggggaggctactgctgggaggatgggtggccttccagtaggcctccagatagtcggcaaggtgctcacaggcatcctcaagctggttctcatccaagatcacatcgaacagctctggaggacactgagccagtttatcagctgctaccatctggacgttgaggtgtttagcttgagatttccctcgagattttattaacctttgtaaaaccttaggagaagaaatctttacatatactataataggggccaaggaggttttactgagttgagctggatgattaattgtatccgcgtcaaggaccaccaactgcaatgttcttgcaagttcaaaaatcctttcgatttcactctgaacttccgctaagcttgaccttgtgttggatctttctattattgcgtgcttactgggattgtttaataccgagcgtttggcaagcgagatgtcagcggtgacccttgtgatggatatccgcccttcaaatctgtgttttaaaaaatcaaacagcgctttttgcatcatatctgtgacctcgtagcccttcagagaagggcccactaggaccactggtcgcatggaaggtaccacatcatacggaggagtgtgctctgtagtaaaccgccaaaacaagcctgcagttttccactggtcttgttcatctgcagattttgcaccagatgatggaggtgttgattttctggaactaggtactatgtcacccaaactggatgatgaatttcctcctgatttactggagtagaatttcccttgcttggctctctgttcatgctgcagcctcatgttttctagtttgactgggcttggaatgaatccgatttcacagccttcttttaccaatcgccctatccaccagtcattgttaaatttttccttaacatgcagaaaatcttttgcttcgaatgagatggccatgccaggcactggaacatcatcttcatgggccgcactgtagctgacatttgtccgaaccgcaaatgcaacgggctttgtctttgctttttccaactgtgcctgggcctgccgctccgcttctctgcgcactgcctcccggtcctcctccagagatacatcggaatcggatggacggctagtgtaggagtctgccgaaccctggcgaacaaaactatttgaggtagtatcagatgacgtgcttccatcagatcctttaaatctgtttttccttctggctccttttccatatgactgtgcggcggctccgagcgcccccgcgggagccacgttctctagcagttccatctggatctcctgcgccaccgccgccgccgctgtgggaggcgacttggacatgtccctttggaccattggcgaaaagtcggctcggagcgaagcagccagcccccggcggcgggtcccctcctcctcgcccccgcctccccgcgctctgatcggctctgggggccgcccagggctcaggcccggccgttctcggcgcagcgccccgcagcgccccgggactcggcgccctgctgccaggcgctcagtgcgcgggacggggccggggcatcgggcgaagcgagccgctcgggaggcgggacgcgggggcgcggctgcggtgcctgggagaggggagccctcagcggggcagccggggccgggagagcgggcgcagcgcggc

SEQ ID NO: 15350 - RNA, 4472 nt, Homo sapiens
  source 1..4472: mol_type = other RNA
gctgggattacaggcatgagccactgcgcccggctgatttattttgttaaataagttaatgtgcagatctgaagttaggtaattatacacaggcattttcctgggacaaacttcaagtgccaggtacttgcactcttaatactgtcttaccatccagttataactggacaaaatatacacttgagacacggaaaaggtcttagccttaaacatgatgacattgtaagcttcttacagcagtgtaattgaggcatggagataatgtcttcaaggttccccttctgtgtacatgtcttatgtaggataatattcttaacattttattcacttcaagtcaccccattttgccctgatttcttctgaagaacagaaactttggttataagaagcacttctgggttctgacagacagtgaacctgctggagtcggtggtggggaggaatggtaggtaactgggaggtaaacaaacaacaggaacaataggcaaggttagaaattgaagtgggagaagttataaaaatttattttcccacgaaataattccacaagctgtgtaaacatttcttactaaaacaaatactctaacacacaaagattgtacatttccagtgaaacactcacagtaaaattgcctgtattttcactctctaggagcaaaaacaaggaggcagcagatgaatgctttcctagttacctttggcagcaagcttactcacattccctgactgctcaatgggttgttaaagcaacatatagcacaattaattaaatacagagcgaggtgggcagaatgctcgatatcagtctctagtttcttcgttagtcttcagcattccaattcatctcaaccattcagtcactcggtgcacactttcttacatacggacacacacacgtgcatatagcgagttccggctcgtagactccagtgcagtgactagaacagacactagctactaagaatgtgtcacaatcagtgtgaactgtatggagtagaacaacctctggagttttatatttaccataatttatggtggaaattacaaacttacttacaaggatggtataacattcagaattcaaaccttttcaagtcaagcaatcacacatatttacagtatgtacacactttctactagaatgaggataggtgtctagacaatgttattacaaatttcctgaatgtgggcatttctagtccctgtaattcataaagcaaatctgctgacttggcattaagactctaaaatagtgtgatcaaactgatatatatatatattatatatataataagaaggtgtttgtttgcagaaataacatttacaaactgtctatacagtacacagtactagtacatagaaaatagattctaactttatgatcccctttgtgtaaggcaagactgaatctgtccccaaatttagtcagccagaggtacaagcaagaaacagtggtccatgaatgaatatgcaaatcagatgcctgcgtattaacgtattaaaaatctggagaaacaagaaattccactttttatctgtgctgattctggcttgttggatacatcaactacatttcttaaaacactaacatcacctgggtggcaacagattttgttcaagtggcagctacccaaaacagtttttgaagagtccagtatgcaaccggaggactgcagccataccaggccaatttatgtagcacttacaaaagaaaaagtatctcaatactctatccatgctattgctattcaagcaacagcaataatacaaaatattacaagacagatcacatatgattgcagtgtagaccccaaagactttgttttggggatgctgttagttatacaagacttcaaaaaaaaaaaaaaaaaaacacaaacgggcaaaactcattggcggatgtaaacatccctgttccactccccagcctcattccgtttttttgatatcacttctccatccttttcacagtagcgatccttggatttatgacggctgcgctgcttgttgcactcgttgtggtcctgctctcgatccacgtcccgggaacggtgccgggactccctgtgtctgtggtcactgctcccgtgggtctcgtctctgtggttgtggtcacggtgtgaggcatagtggtccacgtggtcatgggaataatcttcctttggctctacgtaggcagagtctcgactctcctgggtttccgagtcaaatgtctcttgcctggagaggccgcgacttgtcccactgcgatggttgtggtgtggggctgaggaggaagagcggtgctgggatttcttgactggttccacactaggttcttcttcagcttgggaagcagaacggataggagcggagcgatcagtcctctgatcaccttgagaaccctgtgaattagaggctagggtggggctaagaggcagacttgaagtggctaatgtacggctaaggagagggttggggaggctactgctgggaggatgggtggccttccagtaggcctccagatagtcggcaaggtgctcacaggcatcctcaagctggttctcatccaagatcacatcgaacagctctggaggacactgagccagtttatcagctgctaccatctggacgttgaggtgtttagcttgagatttccctcgagattttattaacctttgtaaaaccttaggagaagaaatctttacatatactataataggggccaaggaggttttactgagttgagctggatgattaattgtatccgcgtcaaggaccaccaactgcaatgttcttgcaagttcaaaaatcctttcgatttcactctgaacttccgctaagcttgaccttgtgttggatctttctattattgcgtgcttactgggattgtttaataccgagcgtttggcaagcgagatgtcagcggtgacccttgtgatggatatccgcccttcaaatctgtgttttaaaaaatcaaacagcgctttttgcatcatatctgtgacctcgtagcccttcagagaagggcccactaggaccactggtcgcatggaaggtaccacatcatacggaggagtgtgctctgtagtaaaccgccaaaacaagcctgcagttttccactggtcttgttcatctgcagattttgcaccagatgatggaggtgttgattttctggaactaggtactatgtcacccaaactggatgatgaatttcctcctgatttactggagtagaatttcccttgcttggctctctgttcatgctgcagcctcatgttttctagtttgactgggcttggaatgaatccgatttcacagccttcttttaccaatcgccctatccaccagtcattgttaaatttttccttaacatgcagaaaatcttttgcttcgaatgagatggccatgccaggcactggaacatcatcttcatgggccgcactgtagctgacatttgtccgaaccgcaaatgcaacgggctttgtctttgctttttccaactgtgcctgggcctgccgctccgcttctctgcgcactgcctcccggtcctcctccagagatacatcggaatcggatggacggctagtgtaggagtctgccgaaccctggcgaacaaaactatttgaggtagtatcagatgacgtgcttccatcagatcctttaaatctgtttttccttctggctccttttccatatgagatcttcagcaggtccagtccactcccctgattcatgtctctccatgtgcctctcccgggaaggggcgaggagggccagctggagcaacccgggagaagtctgggaggactggcaggtctcccccgcccttccccactggcttttcggaagcagagaaaaatggaagccgaggcagagccaggaaaaggcgcaaaggggcagggtccccggcgccaggagaggagcagagggtgggcaggcgacgaggggaggaggtgcgaggctagagatccctgcagtggaggcgccgggagaacccgaggtcggtgccctgcccggcggctcacaaaggaaggagaaggcgccgcgctctcgctacctgtgcggcggctccgagcgcccccgcgggagccacgttctctagcagttccatctggatctcctgcgccaccgccgccgccgctgtgggaggcgacttggacatgtccctttggaccattggcgaaaagtcggctcggagcgaagcagccagcccccggcggcgggtcccctcctcctcgcccccgcctccccgcgctctgatcggctctgggggccgcccagggctcaggcccggccgttctcggcgcagcgccccgcagcgccccgggactcggcgccctgctgccaggcgctcagtgcgcgggacggggccggggcatcgggcgaagcgagccgctcgggaggcgggacgcgggggcgcggctgcggtgcctgggagaggggagccctcagcggggcagccggggccgggagagcgggcgcagcgcggc

SEQ ID NO: 15351 - RNA, 4040 nt, Homo sapiens
  source 1..4040: mol_type = other RNA
gctgggattacaggcatgagccactgcgcccggctgatttattttgttaaataagttaatgtgcagatctgaagttaggtaattatacacaggcattttcctgggacaaacttcaagtgccaggtacttgcactcttaatactgtcttaccatccagttataactggacaaaatatacacttgagacacggaaaaggtcttagccttaaacatgatgacattgtaagcttcttacagcagtgtaattgaggcatggagataatgtcttcaaggttccccttctgtgtacatgtcttatgtaggataatattcttaacattttattcacttcaagtcaccccattttgccctgatttcttctgaagaacagaaactttggttataagaagcacttctgggttctgacagacagtgaacctgctggagtcggtggtggggaggaatggtaggtaactgggaggtaaacaaacaacaggaacaataggcaaggttagaaattgaagtgggagaagttataaaaatttattttcccacgaaataattccacaagctgtgtaaacatttcttactaaaacaaatactctaacacacaaagattgtacatttccagtgaaacactcacagtaaaattgcctgtattttcactctctaggagcaaaaacaaggaggcagcagatgaatgctttcctagttacctttggcagcaagcttactcacattccctgactgctcaatgggttgttaaagcaacatatagcacaattaattaaatacagagcgaggtgggcagaatgctcgatatcagtctctagtttcttcgttagtcttcagcattccaattcatctcaaccattcagtcactcggtgcacactttcttacatacggacacacacacgtgcatatagcgagttccggctcgtagactccagtgcagtgactagaacagacactagctactaagaatgtgtcacaatcagtgtgaactgtatggagtagaacaacctctggagttttatatttaccataatttatggtggaaattacaaacttacttacaaggatggtataacattcagaattcaaaccttttcaagtcaagcaatcacacatatttacagtatgtacacactttctactagaatgaggataggtgtctagacaatgttattacaaatttcctgaatgtgggcatttctagtccctgtaattcataaagcaaatctgctgacttggcattaagactctaaaatagtgtgatcaaactgatatatatatatattatatatataataagaaggtgtttgtttgcagaaataacatttacaaactgtctatacagtacacagtactagtacatagaaaatagattctaactttatgatcccctttgtgtaaggcaagactgaatctgtccccaaatttagtcagccagaggtacaagcaagaaacagtggtccatgaatgaatatgcaaatcagatgcctgcgtattaacgtattaaaaatctggagaaacaagaaattccactttttatctgtgctgattctggcttgttggatacatcaactacatttcttaaaacactaacatcacctgggtggcaacagattttgttcaagtggcagctacccaaaacagtttttgaagagtccagtatgcaaccggaggactgcagccataccaggccaatttatgtagcacttacaaaagaaaaagtatctcaatactctatccatgctattgctattcaagcaacagcaataatacaaaatattacaagacagatcacatatgattgcagtgtagaccccaaagactttgttttggggatgctgttagttatacaagacttcaaaaaaaaaaaaaaaaaaacacaaacgggcaaaactcattggcggatgtaaacatccctgttccactccccagcctcattccgtttttttgatatcacttctccatccttttcacagtagcgatccttggatttatgacggctgcgctgcttgttgcactcgttgtggtcctgctctcgatccacgtcccgggaacggtgccgggactccctgtgtctgtggtcactgctcccgtgggtctcgtctctgtggttgtggtcacggtgtgaggcatagtggtccacgtggtcatgggaataatcttcctttggctctacgtaggcagagtctcgactctcctgggtttccgagtcaaatgtctcttgcctggagaggccgcgacttgtcccactgcgatggttgtggtgtggggctgaggaggaagagcggtgctgggatttcttgactggttccacactaggttcttcttcagcttgggaagcagaacggataggagcggagcgatcagtcctctgatcaccttgagaaccctgtgaattagaggctagggtggggctaagaggcagacttgaagtggctaatgtacggctaaggagagggttggggaggctactgctgggaggatgggtggccttccagtaggcctccagatagtcggcaaggtgctcacaggcatcctcaagctggttctcatccaagatcacatcgaacagctctggaggacactgagccagtttatcagctgctaccatctggacgttgaggtgtttagcttgagatttccctcgagattttattaacctttgtaaaaccttaggagaagaaatctttacatatactataataggggccaaggaggttttactgagttgagctggatgattaattgtatccgcgtcaaggaccaccaactgcaatgttcttgcaagttcaaaaatcctttcgatttcactctgaacttccgctaagcttgaccttgtgttggatctttctattattgcgtgcttactgggattgtttaataccgagcgtttggcaagcgagatgtcagcggtgacccttgtgatggatatccgcccttcaaatctgtgttttaaaaaatcaaacagcgctttttgcatcatatctgtgacctcgtagcccttcagagaagggcccactaggaccactggtcgcatggaaggtaccacatcatacggaggagtgtgctctgtagtaaaccgccaaaacaagcctgcagttttccactggtcttgttcatctgcagattttgcaccgatttctgcttctgcttagcagatgatggaggtgttgattttctggaactaggtactatgtcacccaaactggatgatgaatttcctcctgatttactggagtagaatttcccttgcttggctctctgttcatgctgcagcctcatgttttctagtttgactgggcttggaatgaatccgatttcacagccttcttttaccaatcgccctatccaccagtcattgttaaatttttccttaacatgcagaaaatcttttgcttcgaatgagatggccatgccaggcactggaacatcatcttcatgggccgcactgtagctgacatttgtccgaaccgcaaatgcaacgggctttgtctttgctttttccaactgtgcctgggcctgccgctccgcttctctgcgcactgcctcccggtcctcctccagagatacatcggaatcggatggacggctagtgtaggagtctgccgaaccacagatatcagaattcttcagccttcctcccttggctcttttcagaagcctgatccaggtggccttcatgagccagacagcgcctttatcgtccgcagctgcagccccgggcacaggttctcagtgcgcgctgagccccggagaaccccagctcctttcctatccatgctctgggcaagcccctgttctccgtccctttctgcctccggggctttcactccctgccccagaggactcccatccagggagattcttattttcccattccaggaggggctgaaaacacacactcgagtgctttatattgctttaaaaataaagaagacaagtgcattcaaaagccgagcatcaactcgttctaaacttaatgcatctcataaccctaaacattctcttccctgcgctcaaattgttaaaagaaattagttgtaaa

SEQ ID NO: 15352 - RNA, 3997 nt, Homo sapiens
  source 1..3997: mol_type = other RNA
gctgggattacaggcatgagccactgcgcccggctgatttattttgttaaataagttaatgtgcagatctgaagttaggtaattatacacaggcattttcctgggacaaacttcaagtgccaggtacttgcactcttaatactgtcttaccatccagttataactggacaaaatatacacttgagacacggaaaaggtcttagccttaaacatgatgacattgtaagcttcttacagcagtgtaattgaggcatggagataatgtcttcaaggttccccttctgtgtacatgtcttatgtaggataatattcttaacattttattcacttcaagtcaccccattttgccctgatttcttctgaagaacagaaactttggttataagaagcacttctgggttctgacagacagtgaacctgctggagtcggtggtggggaggaatggtaggtaactgggaggtaaacaaacaacaggaacaataggcaaggttagaaattgaagtgggagaagttataaaaatttattttcccacgaaataattccacaagctgtgtaaacatttcttactaaaacaaatactctaacacacaaagattgtacatttccagtgaaacactcacagtaaaattgcctgtattttcactctctaggagcaaaaacaaggaggcagcagatgaatgctttcctagttacctttggcagcaagcttactcacattccctgactgctcaatgggttgttaaagcaacatatagcacaattaattaaatacagagcgaggtgggcagaatgctcgatatcagtctctagtttcttcgttagtcttcagcattccaattcatctcaaccattcagtcactcggtgcacactttcttacatacggacacacacacgtgcatatagcgagttccggctcgtagactccagtgcagtgactagaacagacactagctactaagaatgtgtcacaatcagtgtgaactgtatggagtagaacaacctctggagttttatatttaccataatttatggtggaaattacaaacttacttacaaggatggtataacattcagaattcaaaccttttcaagtcaagcaatcacacatatttacagtatgtacacactttctactagaatgaggataggtgtctagacaatgttattacaaatttcctgaatgtgggcatttctagtccctgtaattcataaagcaaatctgctgacttggcattaagactctaaaatagtgtgatcaaactgatatatatatatattatatatataataagaaggtgtttgtttgcagaaataacatttacaaactgtctatacagtacacagtactagtacatagaaaatagattctaactttatgatcccctttgtgtaaggcaagactgaatctgtccccaaatttagtcagccagaggtacaagcaagaaacagtggtccatgaatgaatatgcaaatcagatgcctgcgtattaacgtattaaaaatctggagaaacaagaaattccactttttatctgtgctgattctggcttgttggatacatcaactacatttcttaaaacactaacatcacctgggtggcaacagattttgttcaagtggcagctacccaaaacagtttttgaagagtccagtatgcaaccggaggactgcagccataccaggccaatttatgtagcacttacaaaagaaaaagtatctcaatactctatccatgctattgctattcaagcaacagcaataatacaaaatattacaagacagatcacatatgattgcagtgtagaccccaaagactttgttttggggatgctgttagttatacaagacttcaaaaaaaaaaaaaaaaaaacacaaacgggcaaaactcattggcggatgtaaacatccctgttccactccccagcctcattccgtttttttgatatcacttctccatccttttcacagtagcgatccttggatttatgacggctgcgctgcttgttgcactcgttgtggtcctgctctcgatccacgtcccgggaacggtgccgggactccctgtgtctgtggtcactgctcccgtgggtctcgtctctgtggttgtggtcacggtgtgaggcatagtggtccacgtggtcatgggaataatcttcctttggctctacgtaggcagagtctcgactctcctgggtttccgagtcaaatgtctcttgcctggagaggccgcgacttgtcccactgcgatggttgtggtgtggggctgaggaggaagagcggtgctgggatttcttgactggttccacactaggttcttcttcagcttgggaagcagaacggataggagcggagcgatcagtcctctgatcaccttgagaaccctgtgaattagaggctagggtggggctaagaggcagacttgaagtggctaatgtacggctaaggagagggttggggaggctactgctgggaggatgggtggccttccagtaggcctccagatagtcggcaaggtgctcacaggcatcctcaagctggttctcatccaagatcacatcgaacagctctggaggacactgagccagtttatcagctgctaccatctggacgttgaggtgtttagcttgagatttccctcgagattttattaacctttgtaaaaccttaggagaagaaatctttacatatactataataggggccaaggaggttttactgagttgagctggatgattaattgtatccgcgtcaaggaccaccaactgcaatgttcttgcaagttcaaaaatcctttcgatttcactctgaacttccgctaagcttgaccttgtgttggatctttctattattgcgtgcttactgggattgtttaataccgagcgtttggcaagcgagatgtcagcggtgacccttgtgatggatatccgcccttcaaatctgtgttttaaaaaatcaaacagcgctttttgcatcatatctgtgacctcgtagcccttcagagaagggcccactaggaccactggtcgcatggaaggtaccacatcatacggaggagtgtgctctgtagtaaaccgccaaaacaagcctgcagttttccactggtcttgttcatctgcagattttgcaccgatttctgcttctgcttagcagatgatggaggtgttgattttctggaactaggtactatgtcacccaaactggatgatgaatttcctcctgatttactggagtagaatttcccttgcttggctctctgttcatgctgcagcctcatgttttctagtttgactgggcttggaatgaatccgatttcacagccttcttttaccaatcgccctatccaccagtcattgttaaatttttccttaacatgcagaaaatcttttgcttcgaatgagatggccatgccaggcactggaacatcatcttcatgggccgcactgtagctgacatttgtccgaaccgcaaatgcaacgggctttgtctttgctttttccaactgtgcctgggcctgccgctccgcttctctgcgcactgcctcccggtcctcctccagagatacatcggaatcggatggacggctagtgtaggagtctgccgaaccctggcgaacaaaactatttgaggtagtatcagatgacgtgcttccatcagatcctttaaatctgtttttccttctggctccttttccatatgactgtgcggcggctccgagcgcccccgcgggagccacgttctctagcagttccatctggatctcctgcgccaccgccgccgccgctgtgggaggcgacttggacatgtccctttggaccattggcgaaaagtcggctcggagcgaagcagccagcccccggcggcgggtcccctcctcctcgcccccgcctccccgcgctctgatcggctctgggggccgcccagggctcaggcccggccgttctcggcgcagcgccccgcagcgccccgggactcggcgccctgctgccaggcgctc

SEQ ID NO: 15353 - RNA, 3127 nt, Homo sapiens
  source 1..3127: mol_type = other RNA
gctgggattacaggcatgagccactgcgcccggctgatttattttgttaaataagttaatgtgcagatctgaagttaggtaattatacacaggcattttcctgggacaaacttcaagtgccaggtacttgcactcttaatactgtcttaccatccagttataactggacaaaatatacacttgagacacggaaaaggtcttagccttaaacatgatgacattgtaagcttcttacagcagtgtaattgaggcatggagataatgtcttcaaggttccccttctgtgtacatgtcttatgtaggataatattcttaacattttattcacttcaagtcaccccattttgccctgatttcttctgaagaacagaaactttggttataagaagcacttctgggttctgacagacagtgaacctgctggagtcggtggtggggaggaatggtaggtaactgggaggtaaacaaacaacaggaacaataggcaaggttagaaattgaagtgggagaagttataaaaatttattttcccacgaaataattccacaagctgtgtaaacatttcttactaaaacaaatactctaacacacaaagattgtacatttccagtgaaacactcacagtaaaattgcctgtattttcactctctaggagcaaaaacaaggaggcagcagatgaatgctttcctagttacctttggcagcaagcttactcacattccctgactgctcaatgggttgttaaagcaacatatagcacaattaattaaatacagagcgaggtgggcagaatgctcgatatcagtctctagtttcttcgttagtcttcagcattccaattcatctcaaccattcagtcactcggtgcacactttcttacatacggacacacacacgtgcatatagcgagttccggctcgtagactccagtgcagtgactagaacagacactagctactaagaatgtgtcacaatcagtgtgaactgtatggagtagaacaacctctggagttttatatttaccataatttatggtggaaattacaaacttacttacaaggatggtataacattcagaattcaaaccttttcaagtcaagcaatcacacatatttacagtatgtacacactttctactagaatgaggataggtgtctagacaatgttattacaaatttcctgaatgtgggcatttctagtccctgtaattcataaagcaaatctgctgacttggcattaagactctaaaatagtgtgatcaaactgatatatatatatattatatatataataagaaggtgtttgtttgcagaaataacatttacaaactgtctatacagtacacagtactagtacatagaaaatagattctaactttatgatcccctttgtgtaaggcaagactgaatctgtccccaaatttagtcagccagaggtacaagcaagaaacagtggtccatgaatgaatatgcaaatcagatgcctgcgtattaacgtattaaaaatctggagaaacaagaaattccactttttatctgtgctgattctggcttgttggatacatcaactacatttcttaaaacactaacatcacctgggtggcaacagattttgttcaagtggcagctacccaaaacagtttttgaagagtccagtatgcaaccggaggactgcagccataccaggccaatttatgtagcacttacaaaagaaaaagtatctcaatactctatccatgctattgctattcaagcaacagcaataatacaaaatattacaagacagatcacatatgattgcagtgtagaccccaaagactttgttttggggatgctgttagttatacaagacttcaaaaaaaaaaaaaaaaaaacacaaacgggcaaaactcattggcggatgtaaacatccctgttccactccccagcctcattccgtttttttgatatcacttctccatccttttcacagtagcgatccttggatttatgacggctgcgctgcttgttgcactcgttgtggtcctgctctcgatccacgtcccgggaacggtgccgggactccctgtgtctgtggtcactgctcccgtgggtctcgtctctgtggttgtggtcacggtgtgaggcatagtggtccacgtggtcatgggaataatcttcctttggctctacgtaggcagagtctcgactctcctgggtttccgagtcaaatgtctcttgcctggagaggccgcgacttgtcccactgcgatggttgtggtgtggggctgaggaggaagagcggtgctgggatttcttgactggttccacactaggttcttcttcagcttgggaagcagaacggataggagcggagcgatcagtcctctgatcaccttgagaaccctgtgaattagaggctagggtggggctaagaggcagacttgaagtggctaatgtacggctaaggagagggttggggaggctactgctgggaggatgggtggccttccagtaggcctccagatagtcggcaaggtgctcacaggcatcctcaagctggttctcatccaagatcacatcgaacagctctggaggacactgagccagtttatcagctgctaccatctggacgttgaggtgtttagcttgagatttccctcgagattttattaacctttgtaaaaccttaggagaagaaatctttacatatactataataggggccaaggaggttttactgagttgagctggatgattaattgtatccgcgtcaaggaccaccaactgcaatgttcttgcaagttcaaaaatcctttcgatttcactctgaacttccgctaagcttgaccttgtgttggatctttctattattgcgtgcttactgggattgtttaataccgagcgtttggcaagcgagatgtcagcggtgacccttgtgatggatatccgcccttcaaatctgtgttttaaaaaatcaaacagcgctttttgcatcatatctgtgacctcgtagcccttcagagaagggcccactaggaccactggtcgcatggaaggtaccacatcatacggaggagtgtgctctgtcagatgatggaggtgttgattttctggaactaggtactatgtcacccaaactggatgat

SEQ ID NO: 15354 - RNA, 4071 nt, Homo sapiens
  source 1..4071: mol_type = other RNA
gctgggattacaggcatgagccactgcgcccggctgatttattttgttaaataagttaatgtgcagatctgaagttaggtaattatacacaggcattttcctgggacaaacttcaagtgccaggtacttgcactcttaatactgtcttaccatccagttataactggacaaaatatacacttgagacacggaaaaggtcttagccttaaacatgatgacattgtaagcttcttacagcagtgtaattgaggcatggagataatgtcttcaaggttccccttctgtgtacatgtcttatgtaggataatattcttaacattttattcacttcaagtcaccccattttgccctgatttcttctgaagaacagaaactttggttataagaagcacttctgggttctgacagacagtgaacctgctggagtcggtggtggggaggaatggtaggtaactgggaggtaaacaaacaacaggaacaataggcaaggttagaaattgaagtgggagaagttataaaaatttattttcccacgaaataattccacaagctgtgtaaacatttcttactaaaacaaatactctaacacacaaagattgtacatttccagtgaaacactcacagtaaaattgcctgtattttcactctctaggagcaaaaacaaggaggcagcagatgaatgctttcctagttacctttggcagcaagcttactcacattccctgactgctcaatgggttgttaaagcaacatatagcacaattaattaaatacagagcgaggtgggcagaatgctcgatatcagtctctagtttcttcgttagtcttcagcattccaattcatctcaaccattcagtcactcggtgcacactttcttacatacggacacacacacgtgcatatagcgagttccggctcgtagactccagtgcagtgactagaacagacactagctactaagaatgtgtcacaatcagtgtgaactgtatggagtagaacaacctctggagttttatatttaccataatttatggtggaaattacaaacttacttacaaggatggtataacattcagaattcaaaccttttcaagtcaagcaatcacacatatttacagtatgtacacactttctactagaatgaggataggtgtctagacaatgttattacaaatttcctgaatgtgggcatttctagtccctgtaattcataaagcaaatctgctgacttggcattaagactctaaaatagtgtgatcaaactgatatatatatatattatatatataataagaaggtgtttgtttgcagaaataacatttacaaactgtctatacagtacacagtactagtacatagaaaatagattctaactttatgatcccctttgtgtaaggcaagactgaatctgtccccaaatttagtcagccagaggtacaagcaagaaacagtggtccatgaatgaatatgcaaatcagatgcctgcgtattaacgtattaaaaatctggagaaacaagaaattccactttttatctgtgctgattctggcttgttggatacatcaactacatttcttaaaacactaacatcacctgggtggcaacagattttgttcaagtggcagctacccaaaacagtttttgaagagtccagtatgcaaccggaggactgcagccataccaggccaatttatgtagcacttacaaaagaaaaagtatctcaatactctatccatgctattgctattcaagcaacagcaataatacaaaatattacaagacagatcacatatgattgcagtgtagaccccaaagactttgttttggggatgctgttagttatacaagacttcaaaaaaaaaaaaaaaaaaacacaaacgggcaaaactcattggcggatgtaaacatccctgttccactccccagcctcattccgtttttttgatatcacttctccatccttttcacagtagcgatccttggatttatgacggctgcgctgcttgttgcactcgttgtggtcctgctctcgatccacgtcccgggaacggtgccgggactccctgtgtctgtggtcactgctcccgtgggtctcgtctctgtggttgtggtcacggtgtgaggcatagtggtccacgtggtcatgggaataatcttcctttggctctacgtaggcagagtctcgactctcctgggtttccgagtcaaatgtctcttgcctggagaggccgcgacttgtcccactgcgatggttgtggtgtggggctgaggaggaagagcggtgctgggatttcttgactggttccacactaggttcttcttcagcttgggaagcagaacggataggagcggagcgatcagtcctctgatcaccttgagaaccctgtgaattagaggctagggtggggctaagaggcagacttgaagtggctaatgtacggctaaggagagggttggggaggctactgctgggaggatgggtggccttccagtaggcctccagatagtcggcaaggtgctcacaggcatcctcaagctggttctcatccaagatcacatcgaacagctctggaggacactgagccagtttatcagctgctaccatctggacgttgaggtgtttagcttgagatttccctcgagattttattaacctttgtaaaaccttaggagaagaaatctttacatatactataataggggccaaggaggttttactgagttgagctggatgattaattgtatccgcgtcaaggaccaccaactgcaatgttcttgcaagttcaaaaatcctttcgatttcactctgaacttccgctaagcttgaccttgtgttggatctttctattattgcgtgcttactgggattgtttaataccgagcgtttggcaagcgagatgtcagcggtgacccttgtgatggatatccgcccttcaaatctgtgttttaaaaaatcaaacagcgctttttgcatcatatctgtgacctcgtagcccttcagagaagggcccactaggaccactggtcgcatggaaggtaccacatcatacggaggagtgtgctctgtcgatttctgcttctgcttagcagatgatggaggtgttgattttctggaactaggtactatgtcacccaaactggatgatgaatttcctcctgatttactggagtagaatttcccttgcttggctctctgttcatgctgcagcctcatgttttctagtttgactgggcttggaatgaatccgatttcacagccttcttttaccaatcgccctatccaccagtcattgttaaatttttccttaacatgcagaaaatcttttgcttcgaatgagatggccatgccaggcactggaacatcatcttcatgggccgcactgtagctgacatttgtccgaaccgcaaatgcaacgggctttgtctttgctttttccaactgtgcctgggcctgccgctccgcttctctgcgcactgcctcccggtcctcctccagagatacatcggaatcggatggacggctagtgtaggagtctgccgaaccacagatatcagaattcttcagccttcctcccttggctcttttcagaagcctgatccaggtggccttcatgagccagacagcgcctttatcgtccgcagctgcagccccgggcacaggttctcagtgcgcgctgagccccggagaaccccagctcctttcctatccatgctctgggcaagcccctgttctccgtccctttctgcctccggggctttcactccctgccccagaggactcccatccagggagattcttattttcccattccaggaggggctgaaaacacacactcgagtgctttatattgctttaaaaataaagaagacaagtgcattcaaaagccgagcatcaactcgttctaaacttaatgcatctcataaccctaaacattctcttccctgcgctcaaattgttaaaagaaattagttgtaaaagaatcgcagaaaaaaaaaaaaaaaaactagtgcaaaaacgtatgcagtgacatttgcaagtgcaaagttcaagccttatctttggagatctc

SEQ ID NO: 15355 - RNA, 4141 nt, Homo sapiens
  source 1..4141: mol_type = other RNA
gctgggattacaggcatgagccactgcgcccggctgatttattttgttaaataagttaatgtgcagatctgaagttaggtaattatacacaggcattttcctgggacaaacttcaagtgccaggtacttgcactcttaatactgtcttaccatccagttataactggacaaaatatacacttgagacacggaaaaggtcttagccttaaacatgatgacattgtaagcttcttacagcagtgtaattgaggcatggagataatgtcttcaaggttccccttctgtgtacatgtcttatgtaggataatattcttaacattttattcacttcaagtcaccccattttgccctgatttcttctgaagaacagaaactttggttataagaagcacttctgggttctgacagacagtgaacctgctggagtcggtggtggggaggaatggtaggtaactgggaggtaaacaaacaacaggaacaataggcaaggttagaaattgaagtgggagaagttataaaaatttattttcccacgaaataattccacaagctgtgtaaacatttcttactaaaacaaatactctaacacacaaagattgtacatttccagtgaaacactcacagtaaaattgcctgtattttcactctctaggagcaaaaacaaggaggcagcagatgaatgctttcctagttacctttggcagcaagcttactcacattccctgactgctcaatgggttgttaaagcaacatatagcacaattaattaaatacagagcgaggtgggcagaatgctcgatatcagtctctagtttcttcgttagtcttcagcattccaattcatctcaaccattcagtcactcggtgcacactttcttacatacggacacacacacgtgcatatagcgagttccggctcgtagactccagtgcagtgactagaacagacactagctactaagaatgtgtcacaatcagtgtgaactgtatggagtagaacaacctctggagttttatatttaccataatttatggtggaaattacaaacttacttacaaggatggtataacattcagaattcaaaccttttcaagtcaagcaatcacacatatttacagtatgtacacactttctactagaatgaggataggtgtctagacaatgttattacaaatttcctgaatgtgggcatttctagtccctgtaattcataaagcaaatctgctgacttggcattaagactctaaaatagtgtgatcaaactgatatatatatatattatatatataataagaaggtgtttgtttgcagaaataacatttacaaactgtctatacagtacacagtactagtacatagaaaatagattctaactttatgatcccctttgtgtaaggcaagactgaatctgtccccaaatttagtcagccagaggtacaagcaagaaacagtggtccatgaatgaatatgcaaatcagatgcctgcgtattaacgtattaaaaatctggagaaacaagaaattccactttttatctgtgctgattctggcttgttggatacatcaactacatttcttaaaacactaacatcacctgggtggcaacagattttgttcaagtggcagctacccaaaacagtttttgaagagtccagtatgcaaccggaggactgcagccataccaggccaatttatgtagcacttacaaaagaaaaagtatctcaatactctatccatgctattgctattcaagcaacagcaataatacaaaatattacaagacagatcacatatgattgcagtgtagaccccaaagactttgttttggggatgctgttagttatacaagacttcaaaaaaaaaaaaaaaaaaacacaaacgggcaaaactcattggcggatgtaaacatccctgttccactccccagcctcattccgtttttttgatatcacttctccatccttttcacagtagcgatccttggatttatgacggctgcgctgcttgttgcactcgttgtggtcctgctctcgatccacgtcccgggaacggtgccgggactccctgtgtctgtggtcactgctcccgtgggtctcgtctctgtggttgtggtcacggtgtgaggcatagtggtccacgtggtcatgggaataatcttcctttggctctacgtaggcagagtctcgactctcctgggtttccgagtcaaatgtctcttgcctggagaggccgcgacttgtcccactgcgatggttgtggtgtggggctgaggaggaagagcggtgctgggatttcttgactggttccacactaggttcttcttcagcttgggaagcagaacggataggagcggagcgatcagtcctctgatcaccttgagaaccctgtgaattagaggctagggtggggctaagaggcagacttgaagtggctaatgtacggctaaggagagggttggggaggctactgctgggaggatgggtggccttccagtaggcctccagatagtcggcaaggtgctcacaggcatcctcaagctggttctcatccaagatcacatcgaacagctctggaggacactgagccagtttatcagctgctaccatctggacgttgaggtgtttagcttgagatttccctcgagattttattaacctttgtaaaaccttaggagaagaaatctttacatatactataataggggccaaggaggttttactgagttgagctggatgattaattgtatccgcgtcaaggaccaccaactgcaatgttcttgcaagttcaaaaatcctttcgatttcactctgaacttccgctaagcttgaccttgtgttggatctttctattattgcgtgcttactgggattgtttaataccgagcgtttggcaagcgagatgtcagcggtgacccttgtgatggatatccgcccttcaaatctgtgttttaaaaaatcaaacagcgctttttgcatcatatctgtgacctcgtagcccttcagagaagggcccactaggaccactggtcgcatggaaggtaccacatcatacggaggagtgtgctctgtcgatttctgcttctgcttagcagatgatggaggtgttgattttctggaactaggtactatgtcacccaaactggatgatgaatttcctcctgatttactggagtagaatttcccttgcttggctctctgttcatgctgcagcctcatgttttctagtttgactgggcttggaatgaatccgatttcacagccttcttttaccaatcgccctatccaccagtcattgttaaatttttccttaacatgcagaaaatcttttgcttcgaatgagatggccatgccaggcactggaacatcatcttcatgggccgcactgtagctgacatttgtccgaaccgcaaatgcaacgggctttgtctttgctttttccaactgtgcctgggcctgccgctccgcttctctgcgcactgcctcccggtcctcctccagagatacatcggaatcggatggacggctagtgtaggagtctgccgaaccataggacacccgtactcgccggcgatgcaccagcccgcagcactgcatgaagagggggcagaacgcagtcagcgtgtggcttcaccaagctgcactgtgccttgtcttctcgtcacagcctcggtccatttcttcccaccttctactcccaggtaagaggcatgagcaaatcacttagcttctgcctcctaggtagtttctaaaaaagccaccgttcctgcaggcatgccaaaactttgttctcccctgtttgtctttttttgggggtggggggcgtaatttgagatcttcttcaagggggtttcctatttgcaaaaatctacaagaagtagcattaattttccggaagtaagtattgctaacacagagttaggactgtccagatcgtcagagtttcttggtgacgcttttacagtagccattctcaactcgggagattttcaaacatctgagtgtcttgcatttcgcgaccctgcagtactctgcttttgaaaagcaggaggcctactcctgctgctgtttatgtgactgcttcttagcacgctgctgttcctgctcccgcggctgctcgcctatgattgccttcttcacaatgc

SEQ ID NO: 15356 - RNA, 4071 nt, Homo sapiens
  source 1..4071: mol_type = other RNA
gctgggattacaggcatgagccactgcgcccggctgatttattttgttaaataagttaatgtgcagatctgaagttaggtaattatacacaggcattttcctgggacaaacttcaagtgccaggtacttgcactcttaatactgtcttaccatccagttataactggacaaaatatacacttgagacacggaaaaggtcttagccttaaacatgatgacattgtaagcttcttacagcagtgtaattgaggcatggagataatgtcttcaaggttccccttctgtgtacatgtcttatgtaggataatattcttaacattttattcacttcaagtcaccccattttgccctgatttcttctgaagaacagaaactttggttataagaagcacttctgggttctgacagacagtgaacctgctggagtcggtggtggggaggaatggtaggtaactgggaggtaaacaaacaacaggaacaataggcaaggttagaaattgaagtgggagaagttataaaaatttattttcccacgaaataattccacaagctgtgtaaacatttcttactaaaacaaatactctaacacacaaagattgtacatttccagtgaaacactcacagtaaaattgcctgtattttcactctctaggagcaaaaacaaggaggcagcagatgaatgctttcctagttacctttggcagcaagcttactcacattccctgactgctcaatgggttgttaaagcaacatatagcacaattaattaaatacagagcgaggtgggcagaatgctcgatatcagtctctagtttcttcgttagtcttcagcattccaattcatctcaaccattcagtcactcggtgcacactttcttacatacggacacacacacgtgcatatagcgagttccggctcgtagactccagtgcagtgactagaacagacactagctactaagaatgtgtcacaatcagtgtgaactgtatggagtagaacaacctctggagttttatatttaccataatttatggtggaaattacaaacttacttacaaggatggtataacattcagaattcaaaccttttcaagtcaagcaatcacacatatttacagtatgtacacactttctactagaatgaggataggtgtctagacaatgttattacaaatttcctgaatgtgggcatttctagtccctgtaattcataaagcaaatctgctgacttggcattaagactctaaaatagtgtgatcaaactgatatatatatatattatatatataataagaaggtgtttgtttgcagaaataacatttacaaactgtctatacagtacacagtactagtacatagaaaatagattctaactttatgatcccctttgtgtaaggcaagactgaatctgtccccaaatttagtcagccagaggtacaagcaagaaacagtggtccatgaatgaatatgcaaatcagatgcctgcgtattaacgtattaaaaatctggagaaacaagaaattccactttttatctgtgctgattctggcttgttggatacatcaactacatttcttaaaacactaacatcacctgggtggcaacagattttgttcaagtggcagctacccaaaacagtttttgaagagtccagtatgcaaccggaggactgcagccataccaggccaatttatgtagcacttacaaaagaaaaagtatctcaatactctatccatgctattgctattcaagcaacagcaataatacaaaatattacaagacagatcacatatgattgcagtgtagaccccaaagactttgttttggggatgctgttagttatacaagacttcaaaaaaaaaaaaaaaaaaacacaaacgggcaaaactcattggcggatgtaaacatccctgttccactccccagcctcattccgtttttttgatatcacttctccatccttttcacagtagcgatccttggatttatgacggctgcgctgcttgttgcactcgttgtggtcctgctctcgatccacgtcccgggaacggtgccgggactccctgtgtctgtggtcactgctcccgtgggtctcgtctctgtggttgtggtcacggtgtgaggcatagtggtccacgtggtcatgggaataatcttcctttggctctacgtaggcagagtctcgactctcctgggtttccgagtcaaatgtctcttgcctggagaggccgcgacttgtcccactgcgatggttgtggtgtggggctgaggaggaagagcggtgctgggatttcttgactggttccacactaggttcttcttcagcttgggaagcagaacggataggagcggagcgatcagtcctctgatcaccttgagaaccctgtgaattagaggctagggtggggctaagaggcagacttgaagtggctaatgtacggctaaggagagggttggggaggctactgctgggaggatgggtggccttccagtaggcctccagatagtcggcaaggtgctcacaggcatcctcaagctggttctcatccaagatcacatcgaacagctctggaggacactgagccagtttatcagctgctaccatctggacgttgaggtgtttagcttgagatttccctcgagattttattaacctttgtaaaaccttaggagaagaaatctttacatatactataataggggccaaggaggttttactgagttgagctggatgattaattgtatccgcgtcaaggaccaccaactgcaatgttcttgcaagttcaaaaatcctttcgatttcactctgaacttccgctaagcttgaccttgtgttggatctttctattattgcgtgcttactgggattgtttaataccgagcgtttggcaagcgagatgtcagcggtgacccttgtgatggatatccgcccttcaaatctgtgttttaaaaaatcaaacagcgctttttgcatcatatctgtgacctcgtagcccttcagagaagggcccactaggaccactggtcgcatggaaggtaccacatcatacggaggagtgtgctctgtcgatttctgcttctgcttagcagatgatggaggtgttgattttctggaactaggtactatgtcacccaaactggatgatgaatttcctcctgatttactggagtagaatttcccttgcttggctctctgttcatgctgcagcctcatgttttctagtttgactgggcttggaatgaatccgatttcacagccttcttttaccaatcgccctatccaccagtcattgttaaatttttccttaacatgcagaaaatcttttgcttcgaatgagatggccatgccaggcactggaacatcatcttcatgggccgcactgtagctgacatttgtccgaaccgcaaatgcaacgggctttgtctttgctttttccaactgtgcctgggcctgccgctccgcttctctgcgcactgcctcccggtcctcctccagagatacatcggaatcggatggacggctagtgtaggagtctgccgaaccctggcgaacaaaactatttgaggtagtatcagatgacgtgcttccatcagatcctttaaatctgtttttccttctggctccttttccatatgactgtgcggcggctccgagcgcccccgcgggagccacgttctctagcagttccatctggatctcctgcgccaccgccgccgccgctgtgggaggcgacttggacatgtccctttggaccattggcgaaaagtcggctcggagcgaagcagccagcccccggcggcgggtcccctcctcctcgcccccgcctccccgcgctctgatcggctctgggggccgcccagggctcaggcccggccgttctcggcgcagcgccccgcagcgccccgggactcggcgccctgctgccaggcgctcagtgcgcgggacggggccggggcatcgggcgaagcgagccgctcgggaggcgggacgcgggggcgcggctgcggtgcctgggagaggggagccctcagcggggcagccggggccgggagagcgggcgcagcgcggc

SEQ ID NO: 15357 - RNA, 4430 nt, Homo sapiens
  source 1..4430: mol_type = other RNA
gctgggattacaggcatgagccactgcgcccggctgatttattttgttaaataagttaatgtgcagatctgaagttaggtaattatacacaggcattttcctgggacaaacttcaagtgccaggtacttgcactcttaatactgtcttaccatccagttataactggacaaaatatacacttgagacacggaaaaggtcttagccttaaacatgatgacattgtaagcttcttacagcagtgtaattgaggcatggagataatgtcttcaaggttccccttctgtgtacatgtcttatgtaggataatattcttaacattttattcacttcaagtcaccccattttgccctgatttcttctgaagaacagaaactttggttataagaagcacttctgggttctgacagacagtgaacctgctggagtcggtggtggggaggaatggtaggtaactgggaggtaaacaaacaacaggaacaataggcaaggttagaaattgaagtgggagaagttataaaaatttattttcccacgaaataattccacaagctgtgtaaacatttcttactaaaacaaatactctaacacacaaagattgtacatttccagtgaaacactcacagtaaaattgcctgtattttcactctctaggagcaaaaacaaggaggcagcagatgaatgctttcctagttacctttggcagcaagcttactcacattccctgactgctcaatgggttgttaaagcaacatatagcacaattaattaaatacagagcgaggtgggcagaatgctcgatatcagtctctagtttcttcgttagtcttcagcattccaattcatctcaaccattcagtcactcggtgcacactttcttacatacggacacacacacgtgcatatagcgagttccggctcgtagactccagtgcagtgactagaacagacactagctactaagaatgtgtcacaatcagtgtgaactgtatggagtagaacaacctctggagttttatatttaccataatttatggtggaaattacaaacttacttacaaggatggtataacattcagaattcaaaccttttcaagtcaagcaatcacacatatttacagtatgtacacactttctactagaatgaggataggtgtctagacaatgttattacaaatttcctgaatgtgggcatttctagtccctgtaattcataaagcaaatctgctgacttggcattaagactctaaaatagtgtgatcaaactgatatatatatatattatatatataataagaaggtgtttgtttgcagaaataacatttacaaactgtctatacagtacacagtactagtacatagaaaatagattctaactttatgatcccctttgtgtaaggcaagactgaatctgtccccaaatttagtcagccagaggtacaagcaagaaacagtggtccatgaatgaatatgcaaatcagatgcctgcgtattaacgtattaaaaatctggagaaacaagaaattccactttttatctgtgctgattctggcttgttggatacatcaactacatttcttaaaacactaacatcacctgggtggcaacagattttgttcaagtggcagctacccaaaacagtttttgaagagtccagtatgcaaccggaggactgcagccataccaggccaatttatgtagcacttacaaaagaaaaagtatctcaatactctatccatgctattgctattcaagcaacagcaataatacaaaatattacaagacagatcacatatgattgcagtgtagaccccaaagactttgttttggggatgctgttagttatacaagacttcaaaaaaaaaaaaaaaaaaacacaaacgggcaaaactcattggcggatgtaaacatccctgttccactccccagcctcattccgtttttttgatatcacttctccatccttttcacagtagcgatccttggatttatgacggctgcgctgcttgttgcactcgttgtggtcctgctctcgatccacgtcccgggaacggtgccgggactccctgtgtctgtggtcactgctcccgtgggtctcgtctctgtggttgtggtcacggtgtgaggcatagtggtccacgtggtcatgggaataatcttcctttggctctacgtaggcagagtctcgactctcctgggtttccgagtcaaatgtctcttgcctggagaggccgcgacttgtcccactgcgatggttgtggtgtggggctgaggaggaagagcggtgctgggatttcttgactggttccacactaggttcttcttcagcttgggaagcagaacggataggagcggagcgatcagtcctctgatcaccttgagaaccctgtgaattagaggctagggtggggctaagaggcagacttgaagtggctaatgtacggctaaggagagggttggggaggctactgctgggaggatgggtggccttccagtaggcctccagatagtcggcaaggtgctcacaggcatcctcaagctggttctcatccaagatcacatcgaacagctctggaggacactgagccagtttatcagctgctaccatctggacgttgaggtgtttagcttgagatttccctcgagattttattaacctttgtaaaaccttaggagaagaaatctttacatatactataataggggccaaggaggttttactgagttgagctggatgattaattgtatccgcgtcaaggaccaccaactgcaatgttcttgcaagttcaaaaatcctttcgatttcactctgaacttccgctaagcttgaccttgtgttggatctttctattattgcgtgcttactgggattgtttaataccgagcgtttggcaagcgagatgtcagcggtgacccttgtgatggatatccgcccttcaaatctgtgttttaaaaaatcaaacagcgctttttgcatcatatctgtgacctcgtagcccttcagagaagggcccactaggaccactggtcgcatggaaggtaccacatcatacggaggagtgtgctctgtcgatttctgcttctgcttagcagatgatggaggtgttgattttctggaactaggtactatgtcacccaaactggatgatgaatttcctcctgatttactggagtagaatttcccttgcttggctctctgttcatgctgcagcctcatgttttctagtttgactgggcttggaatgaatccgatttcacagccttcttttaccaatcgccctatccaccagtcattgttaaatttttccttaacatgcagaaaatcttttgcttcgaatgagatggccatgccaggcactggaacatcatcttcatgggccgcactgtagctgacatttgtccgaaccgcaaatgcaacgggctttgtctttgctttttccaactgtgcctgggcctgccgctccgcttctctgcgcactgcctcccggtcctcctccagagatacatcggaatcggatggacggctagtgtaggagtctgccgaaccctggcgaacaaaactatttgaggtagtatcagatgacgtgcttccatcagatcctttaaatctgtttttccttctggctccttttccatatgagatcttcagcaggtccagtccactcccctgattcatgtctctccatgtgcctctcccgggaaggggcgaggagggccagctggagcaacccgggagaagtctgggaggactggcaggtctcccccgcccttccccactggcttttcggaagcagagaaaaatggaagccgaggcagagccaggaaaaggcgcaaaggggcagggtccccggcgccaggagaggagcagagggtgggcaggcgacgaggggaggaggtgcgaggctagagatccctgcagtggaggcgccgggagaacccgaggtcggtgccctgcccggcggctcacaaaggaaggagaaggcgccgcgctctcgctacctgtgcggcggctccgagcgcccccgcgggagccacgttctctagcagttccatctggatctcctgcgccaccgccgccgccgctgtgggaggcgacttggacatgtccctttggaccattggcgaaaagtcggctcggagcgaagcagccagcccccggcggcgggtcccctcctcctcgcccccgcctccccgcgctctgatcggctctgggggccgcccagggctcaggcccggccgttctcggcgcagcgccccgcagcgccccgggactcggcgccctgctgccaggcgctcagtgcgcgggacggggccggggcatcgggcgaagcgagccgctcgggaggcgggacgcgggggcgcggctgcggtgcctgggagaggggagccctcagcggggcagccggggccgggagagcgggcgcagcgcggc

SEQ ID NO: 15358 - RNA, 4185 nt, Homo sapiens
  source 1..4185: mol_type = other RNA
gctgggattacaggcatgagccactgcgcccggctgatttattttgttaaataagttaatgtgcagatctgaagttaggtaattatacacaggcattttcctgggacaaacttcaagtgccaggtacttgcactcttaatactgtcttaccatccagttataactggacaaaatatacacttgagacacggaaaaggtcttagccttaaacatgatgacattgtaagcttcttacagcagtgtaattgaggcatggagataatgtcttcaaggttccccttctgtgtacatgtcttatgtaggataatattcttaacattttattcacttcaagtcaccccattttgccctgatttcttctgaagaacagaaactttggttataagaagcacttctgggttctgacagacagtgaacctgctggagtcggtggtggggaggaatggtaggtaactgggaggtaaacaaacaacaggaacaataggcaaggttagaaattgaagtgggagaagttataaaaatttattttcccacgaaataattccacaagctgtgtaaacatttcttactaaaacaaatactctaacacacaaagattgtacatttccagtgaaacactcacagtaaaattgcctgtattttcactctctaggagcaaaaacaaggaggcagcagatgaatgctttcctagttacctttggcagcaagcttactcacattccctgactgctcaatgggttgttaaagcaacatatagcacaattaattaaatacagagcgaggtgggcagaatgctcgatatcagtctctagtttcttcgttagtcttcagcattccaattcatctcaaccattcagtcactcggtgcacactttcttacatacggacacacacacgtgcatatagcgagttccggctcgtagactccagtgcagtgactagaacagacactagctactaagaatgtgtcacaatcagtgtgaactgtatggagtagaacaacctctggagttttatatttaccataatttatggtggaaattacaaacttacttacaaggatggtataacattcagaattcaaaccttttcaagtcaagcaatcacacatatttacagtatgtacacactttctactagaatgaggataggtgtctagacaatgttattacaaatttcctgaatgtgggcatttctagtccctgtaattcataaagcaaatctgctgacttggcattaagactctaaaatagtgtgatcaaactgatatatatatatattatatatataataagaaggtgtttgtttgcagaaataacatttacaaactgtctatacagtacacagtactagtacatagaaaatagattctaactttatgatcccctttgtgtaaggcaagactgaatctgtccccaaatttagtcagccagaggtacaagcaagaaacagtggtccatgaatgaatatgcaaatcagatgcctgcgtattaacgtattaaaaatctggagaaacaagaaattccactttttatctgtgctgattctggcttgttggatacatcaactacatttcttaaaacactaacatcacctgggtggcaacagattttgttcaagtggcagctacccaaaacagtttttgaagagtccagtatgcaaccggaggactgcagccataccaggccaatttatgtagcacttacaaaagaaaaagtatctcaatactctatccatgctattgctattcaagcaacagcaataatacaaaatattacaagacagatcacatatgattgcagtgtagaccccaaagactttgttttggggatgctgttagttatacaagacttcaaaaaaaaaaaaaaaaaaacacaaacgggcaaaactcattggcggatgtaaacatccctgttccactccccagcctcattccgtttttttgatatcacttctccatccttttcacagtagcgatccttggatttatgacggctgcgctgcttgttgcactcgttgtggtcctgctctcgatccacgtcccgggaacggtgccgggactccctgtgtctgtggtcactgctcccgtgggtctcgtctctgtggttgtggtcacggtgtgaggcatagtggtccacgtggtcatgggaataatcttcctttggctctacgtaggcagagtctcgactctcctgggtttccgagtcaaatgtctcttgcctggagaggccgcgacttgtcccactgcgatggttgtggtgtggggctgaggaggaagagcggtgctgggatttcttgactggttccacactaggttcttcttcagcttgggaagcagaacggataggagcggagcgatcagtcctctgatcaccttgagaaccctgtgaattagaggctagggtggggctaagaggcagacttgaagtggctaatgtacggctaaggagagggttggggaggctactgctgggaggatgggtggccttccagtaggcctccagatagtcggcaaggtgctcacaggcatcctcaagctggttctcatccaagatcacatcgaacagctctggaggacactgagccagtttatcagctgctaccatctggacgttgaggtgtttagcttgagatttccctcgagattttattaacctttgtaaaaccttaggagaagaaatctttacatatactataataggggccaaggaggttttactgagttgagctggatgattaattgtatccgcgtcaaggaccaccaactgcaatgttcttgcaagttcaaaaatcctttcgatttcactctgaacttccgctaagcttgaccttgtgttggatctttctattattgcgtgcttactgggattgtttaataccgagcgtttggcaagcgagatgtcagcggtgacccttgtgatggatatccgcccttcaaatctgtgttttaaaaaatcaaacagcgctttttgcatcatatctgtgacctcgtagcccttcagagaagggcccactaggaccactggtcgcatggaaggtaccacatcatacggaggagtgtgctctgtcttcttaaagaagggcattcttttctctttggagtggggtgacgttacactgtttgcactgggtttaggggagcggtggtttgctggaatatcattttcttctgcatctaagccagtagcatctatgtctatagcagatgatggaggtgttgattttctggaactaggtactatgtcacccaaactggatgatgaatttcctcctgatttactggagtagaatttcccttgcttggctctctgttcatgctgcagcctcatgttttctagtttgactgggcttggaatgaatccgatttcacagccttcttttaccaatcgccctatccaccagtcattgttaaatttttccttaacatgcagaaaatcttttgcttcgaatgagatggccatgccaggcactggaacatcatcttcatgggccgcactgtagctgacatttgtccgaaccgcaaatgcaacgggctttgtctttgctttttccaactgtgcctgggcctgccgctccgcttctctgcgcactgcctcccggtcctcctccagagatacatcggaatcggatggacggctagtgtaggagtctgccgaaccacagatatcagaattcttcagccttcctcccttggctcttttcagaagcctgatccaggtggccttcatgagccagacagcgcctttatcgtccgcagctgcagccccgggcacaggttctcagtgcgcgctgagccccggagaaccccagctcctttcctatccatgctctgggcaagcccctgttctccgtccctttctgcctccggggctttcactccctgccccagaggactcccatccagggagattcttattttcccattccaggaggggctgaaaacacacactcgagtgctttatattgctttaaaaataaagaagacaagtgcattcaaaagccgagcatcaactcgttctaaacttaatgcatctcataaccctaaacattctcttccctgcgctcaaattgttaaaagaaattagttgtaaaagaatcgcagaaaaaaaaaaaaaaaaactagtgcaaaaacgtatgcagtgacatttgcaagtgcaaagttcaagccttatctttggagatctc

SEQ ID NO: 15359 - RNA, 4255 nt, Homo sapiens
  source 1..4255: mol_type = other RNA
gctgggattacaggcatgagccactgcgcccggctgatttattttgttaaataagttaatgtgcagatctgaagttaggtaattatacacaggcattttcctgggacaaacttcaagtgccaggtacttgcactcttaatactgtcttaccatccagttataactggacaaaatatacacttgagacacggaaaaggtcttagccttaaacatgatgacattgtaagcttcttacagcagtgtaattgaggcatggagataatgtcttcaaggttccccttctgtgtacatgtcttatgtaggataatattcttaacattttattcacttcaagtcaccccattttgccctgatttcttctgaagaacagaaactttggttataagaagcacttctgggttctgacagacagtgaacctgctggagtcggtggtggggaggaatggtaggtaactgggaggtaaacaaacaacaggaacaataggcaaggttagaaattgaagtgggagaagttataaaaatttattttcccacgaaataattccacaagctgtgtaaacatttcttactaaaacaaatactctaacacacaaagattgtacatttccagtgaaacactcacagtaaaattgcctgtattttcactctctaggagcaaaaacaaggaggcagcagatgaatgctttcctagttacctttggcagcaagcttactcacattccctgactgctcaatgggttgttaaagcaacatatagcacaattaattaaatacagagcgaggtgggcagaatgctcgatatcagtctctagtttcttcgttagtcttcagcattccaattcatctcaaccattcagtcactcggtgcacactttcttacatacggacacacacacgtgcatatagcgagttccggctcgtagactccagtgcagtgactagaacagacactagctactaagaatgtgtcacaatcagtgtgaactgtatggagtagaacaacctctggagttttatatttaccataatttatggtggaaattacaaacttacttacaaggatggtataacattcagaattcaaaccttttcaagtcaagcaatcacacatatttacagtatgtacacactttctactagaatgaggataggtgtctagacaatgttattacaaatttcctgaatgtgggcatttctagtccctgtaattcataaagcaaatctgctgacttggcattaagactctaaaatagtgtgatcaaactgatatatatatatattatatatataataagaaggtgtttgtttgcagaaataacatttacaaactgtctatacagtacacagtactagtacatagaaaatagattctaactttatgatcccctttgtgtaaggcaagactgaatctgtccccaaatttagtcagccagaggtacaagcaagaaacagtggtccatgaatgaatatgcaaatcagatgcctgcgtattaacgtattaaaaatctggagaaacaagaaattccactttttatctgtgctgattctggcttgttggatacatcaactacatttcttaaaacactaacatcacctgggtggcaacagattttgttcaagtggcagctacccaaaacagtttttgaagagtccagtatgcaaccggaggactgcagccataccaggccaatttatgtagcacttacaaaagaaaaagtatctcaatactctatccatgctattgctattcaagcaacagcaataatacaaaatattacaagacagatcacatatgattgcagtgtagaccccaaagactttgttttggggatgctgttagttatacaagacttcaaaaaaaaaaaaaaaaaaacacaaacgggcaaaactcattggcggatgtaaacatccctgttccactccccagcctcattccgtttttttgatatcacttctccatccttttcacagtagcgatccttggatttatgacggctgcgctgcttgttgcactcgttgtggtcctgctctcgatccacgtcccgggaacggtgccgggactccctgtgtctgtggtcactgctcccgtgggtctcgtctctgtggttgtggtcacggtgtgaggcatagtggtccacgtggtcatgggaataatcttcctttggctctacgtaggcagagtctcgactctcctgggtttccgagtcaaatgtctcttgcctggagaggccgcgacttgtcccactgcgatggttgtggtgtggggctgaggaggaagagcggtgctgggatttcttgactggttccacactaggttcttcttcagcttgggaagcagaacggataggagcggagcgatcagtcctctgatcaccttgagaaccctgtgaattagaggctagggtggggctaagaggcagacttgaagtggctaatgtacggctaaggagagggttggggaggctactgctgggaggatgggtggccttccagtaggcctccagatagtcggcaaggtgctcacaggcatcctcaagctggttctcatccaagatcacatcgaacagctctggaggacactgagccagtttatcagctgctaccatctggacgttgaggtgtttagcttgagatttccctcgagattttattaacctttgtaaaaccttaggagaagaaatctttacatatactataataggggccaaggaggttttactgagttgagctggatgattaattgtatccgcgtcaaggaccaccaactgcaatgttcttgcaagttcaaaaatcctttcgatttcactctgaacttccgctaagcttgaccttgtgttggatctttctattattgcgtgcttactgggattgtttaataccgagcgtttggcaagcgagatgtcagcggtgacccttgtgatggatatccgcccttcaaatctgtgttttaaaaaatcaaacagcgctttttgcatcatatctgtgacctcgtagcccttcagagaagggcccactaggaccactggtcgcatggaaggtaccacatcatacggaggagtgtgctctgtcttcttaaagaagggcattcttttctctttggagtggggtgacgttacactgtttgcactgggtttaggggagcggtggtttgctggaatatcattttcttctgcatctaagccagtagcatctatgtctatagcagatgatggaggtgttgattttctggaactaggtactatgtcacccaaactggatgatgaatttcctcctgatttactggagtagaatttcccttgcttggctctctgttcatgctgcagcctcatgttttctagtttgactgggcttggaatgaatccgatttcacagccttcttttaccaatcgccctatccaccagtcattgttaaatttttccttaacatgcagaaaatcttttgcttcgaatgagatggccatgccaggcactggaacatcatcttcatgggccgcactgtagctgacatttgtccgaaccgcaaatgcaacgggctttgtctttgctttttccaactgtgcctgggcctgccgctccgcttctctgcgcactgcctcccggtcctcctccagagatacatcggaatcggatggacggctagtgtaggagtctgccgaaccataggacacccgtactcgccggcgatgcaccagcccgcagcactgcatgaagagggggcagaacgcagtcagcgtgtggcttcaccaagctgcactgtgccttgtcttctcgtcacagcctcggtccatttcttcccaccttctactcccaggtaagaggcatgagcaaatcacttagcttctgcctcctaggtagtttctaaaaaagccaccgttcctgcaggcatgccaaaactttgttctcccctgtttgtctttttttgggggtggggggcgtaatttgagatcttcttcaagggggtttcctatttgcaaaaatctacaagaagtagcattaattttccggaagtaagtattgctaacacagagttaggactgtccagatcgtcagagtttcttggtgacgcttttacagtagccattctcaactcgggagattttcaaacatctgagtgtcttgcatttcgcgaccctgcagtactctgcttttgaaaagcaggaggcctactcctgctgctgtttatgtgactgcttcttagcacgctgctgttcctgctcccgcggctgctcgcctatgattgccttcttcacaatgc

SEQ ID NO: 15360 - RNA, 3985 nt, Homo sapiens
  source 1..3985: mol_type = other RNA
gctgggattacaggcatgagccactgcgcccggctgatttattttgttaaataagttaatgtgcagatctgaagttaggtaattatacacaggcattttcctgggacaaacttcaagtgccaggtacttgcactcttaatactgtcttaccatccagttataactggacaaaatatacacttgagacacggaaaaggtcttagccttaaacatgatgacattgtaagcttcttacagcagtgtaattgaggcatggagataatgtcttcaaggttccccttctgtgtacatgtcttatgtaggataatattcttaacattttattcacttcaagtcaccccattttgccctgatttcttctgaagaacagaaactttggttataagaagcacttctgggttctgacagacagtgaacctgctggagtcggtggtggggaggaatggtaggtaactgggaggtaaacaaacaacaggaacaataggcaaggttagaaattgaagtgggagaagttataaaaatttattttcccacgaaataattccacaagctgtgtaaacatttcttactaaaacaaatactctaacacacaaagattgtacatttccagtgaaacactcacagtaaaattgcctgtattttcactctctaggagcaaaaacaaggaggcagcagatgaatgctttcctagttacctttggcagcaagcttactcacattccctgactgctcaatgggttgttaaagcaacatatagcacaattaattaaatacagagcgaggtgggcagaatgctcgatatcagtctctagtttcttcgttagtcttcagcattccaattcatctcaaccattcagtcactcggtgcacactttcttacatacggacacacacacgtgcatatagcgagttccggctcgtagactccagtgcagtgactagaacagacactagctactaagaatgtgtcacaatcagtgtgaactgtatggagtagaacaacctctggagttttatatttaccataatttatggtggaaattacaaacttacttacaaggatggtataacattcagaattcaaaccttttcaagtcaagcaatcacacatatttacagtatgtacacactttctactagaatgaggataggtgtctagacaatgttattacaaatttcctgaatgtgggcatttctagtccctgtaattcataaagcaaatctgctgacttggcattaagactctaaaatagtgtgatcaaactgatatatatatatattatatatataataagaaggtgtttgtttgcagaaataacatttacaaactgtctatacagtacacagtactagtacatagaaaatagattctaactttatgatcccctttgtgtaaggcaagactgaatctgtccccaaatttagtcagccagaggtacaagcaagaaacagtggtccatgaatgaatatgcaaatcagatgcctgcgtattaacgtattaaaaatctggagaaacaagaaattccactttttatctgtgctgattctggcttgttggatacatcaactacatttcttaaaacactaacatcacctgggtggcaacagattttgttcaagtggcagctacccaaaacagtttttgaagagtccagtatgcaaccggaggactgcagccataccaggccaatttatgtagcacttacaaaagaaaaagtatctcaatactctatccatgctattgctattcaagcaacagcaataatacaaaatattacaagacagatcacatatgattgcagtgtagaccccaaagactttgttttggggatgctgttagttatacaagacttcaaaaaaaaaaaaaaaaaaacacaaacgggcaaaactcattggcggatgtaaacatccctgttccactccccagcctcattccgtttttttgatatcacttctccatccttttcacagtagcgatccttggatttatgacggctgcgctgcttgttgcactcgttgtggtcctgctctcgatccacgtcccgggaacggtgccgggactccctgtgtctgtggtcactgctcccgtgggtctcgtctctgtggttgtggtcacggtgtgaggcatagtggtccacgtggtcatgggaataatcttcctttggctctacgtaggcagagtctcgactctcctgggtttccgagtcaaatgtctcttgcctggagaggccgcgacttgtcccactgcgatggttgtggtgtggggctgaggaggaagagcggtgctgggatttcttgactggttccacactaggttcttcttcagcttgggaagcagaacggataggagcggagcgatcagtcctctgatcaccttgagaaccctgtgaattagaggctagggtggggctaagaggcagacttgaagtggctaatgtacggctaaggagagggttggggaggctactgctgggaggatgggtggccttccagtaggcctccagatagtcggcaaggtgctcacaggcatcctcaagctggttctcatccaagatcacatcgaacagctctggaggacactgagccagtttatcagctgctaccatctggacgttgaggtgtttagcttgagatttccctcgagattttattaacctttgtaaaaccttaggagaagaaatctttacatatactataataggggccaaggaggttttactgagttgagctggatgattaattgtatccgcgtcaaggaccaccaactgcaatgttcttgcaagttcaaaaatcctttcgatttcactctgaacttccgctaagcttgaccttgtgttggatctttctattattgcgtgcttactgggattgtttaataccgagcgtttggcaagcgagatgtcagcggtgacccttgtgatggatatccgcccttcaaatctgtgttttaaaaaatcaaacagcgctttttgcatcatatctgtgacctcgtagcccttcagagaagggcccactaggaccactggtcgcatggaaggtaccacatcatacggaggagtgtgctctgtcttcttaaagaagggcattcttttctctttggagtggggtgacgttacactgtttgcactgggtttaggggagcggtggtttgctggaatatcattttcttctgcatctaagccagtagcatctatgtctatagcagatgatggaggtgttgattttctggaactaggtactatgtcacccaaactggatgatgaatttcctcctgatttactggagtagaatttcccttgcttggctctctgttcatgctgcagcctcatgttttctagtttgactgggcttggaatgaatccgatttcacagccttcttttaccaatcgccctatccaccagtcattgttaaatttttccttaacatgcagaaaatcttttgcttcgaatgagatggccatgccaggcactggaacatcatcttcatgggccgcactgtagctgacatttgtccgaaccgcaaatgcaacgggctttgtctttgctttttccaactgtgcctgggcctgccgctccgcttctctgcgcactgcctcccggtcctcctccagagatacatcggaatcggatggacggctagtgtaggagtctgccgaacccacttcagaaggctcatcgtcatcgtagtacatgtttcgtacacacctcgaagtaaattctcagcatgtccgctaagaaatcctttcataggaagttcaagtgcattatgacagtgatacagtttccacagctggaatatagtgatactagtttcccacgcttggcaatgctcttaaaataggctctcagacaccaaaagacaaaaaatgactatttgtaagcacttcaggaaatgatgctctggcaaactgactgaaaattccataaacagccaaaatcagctttttttttttgagacggagtctcgctttgttgcccaggctgg

SEQ ID NO: 15361 - RNA, 3928 nt, Homo sapiens
  source 1..3928: mol_type = other RNA
gctgggattacaggcatgagccactgcgcccggctgatttattttgttaaataagttaatgtgcagatctgaagttaggtaattatacacaggcattttcctgggacaaacttcaagtgccaggtacttgcactcttaatactgtcttaccatccagttataactggacaaaatatacacttgagacacggaaaaggtcttagccttaaacatgatgacattgtaagcttcttacagcagtgtaattgaggcatggagataatgtcttcaaggttccccttctgtgtacatgtcttatgtaggataatattcttaacattttattcacttcaagtcaccccattttgccctgatttcttctgaagaacagaaactttggttataagaagcacttctgggttctgacagacagtgaacctgctggagtcggtggtggggaggaatggtaggtaactgggaggtaaacaaacaacaggaacaataggcaaggttagaaattgaagtgggagaagttataaaaatttattttcccacgaaataattccacaagctgtgtaaacatttcttactaaaacaaatactctaacacacaaagattgtacatttccagtgaaacactcacagtaaaattgcctgtattttcactctctaggagcaaaaacaaggaggcagcagatgaatgctttcctagttacctttggcagcaagcttactcacattccctgactgctcaatgggttgttaaagcaacatatagcacaattaattaaatacagagcgaggtgggcagaatgctcgatatcagtctctagtttcttcgttagtcttcagcattccaattcatctcaaccattcagtcactcggtgcacactttcttacatacggacacacacacgtgcatatagcgagttccggctcgtagactccagtgcagtgactagaacagacactagctactaagaatgtgtcacaatcagtgtgaactgtatggagtagaacaacctctggagttttatatttaccataatttatggtggaaattacaaacttacttacaaggatggtataacattcagaattcaaaccttttcaagtcaagcaatcacacatatttacagtatgtacacactttctactagaatgaggataggtgtctagacaatgttattacaaatttcctgaatgtgggcatttctagtccctgtaattcataaagcaaatctgctgacttggcattaagactctaaaatagtgtgatcaaactgatatatatatatattatatatataataagaaggtgtttgtttgcagaaataacatttacaaactgtctatacagtacacagtactagtacatagaaaatagattctaactttatgatcccctttgtgtaaggcaagactgaatctgtccccaaatttagtcagccagaggtacaagcaagaaacagtggtccatgaatgaatatgcaaatcagatgcctgcgtattaacgtattaaaaatctggagaaacaagaaattccactttttatctgtgctgattctggcttgttggatacatcaactacatttcttaaaacactaacatcacctgggtggcaacagattttgttcaagtggcagctacccaaaacagtttttgaagagtccagtatgcaaccggaggactgcagccataccaggccaatttatgtagcacttacaaaagaaaaagtatctcaatactctatccatgctattgctattcaagcaacagcaataatacaaaatattacaagacagatcacatatgattgcagtgtagaccccaaagactttgttttggggatgctgttagttatacaagacttcaaaaaaaaaaaaaaaaaaacacaaacgggcaaaactcattggcggatgtaaacatccctgttccactccccagcctcattccgtttttttgatatcacttctccatccttttcacagtagcgatccttggatttatgacggctgcgctgcttgttgcactcgttgtggtcctgctctcgatccacgtcccgggaacggtgccgggactccctgtgtctgtggtcactgctcccgtgggtctcgtctctgtggttgtggtcacggtgtgaggcatagtggtccacgtggtcatgggaataatcttcctttggctctacgtaggcagagtctcgactctcctgggtttccgagtcaaatgtctcttgcctggagaggccgcgacttgtcccactgcgatggttgtggtgtggggctgaggaggaagagcggtgctgggatttcttgactggttccacactaggttcttcttcagcttgggaagcagaacggataggagcggagcgatcagtcctctgatcaccttgagaaccctgtgaattagaggctagggtggggctaagaggcagacttgaagtggctaatgtacggctaaggagagggttggggaggctactgctgggaggatgggtggccttccagtaggcctccagatagtcggcaaggtgctcacaggcatcctcaagctggttctcatccaagatcacatcgaacagctctggaggacactgagccagtttatcagctgctaccatctggacgttgaggtgtttagcttgagatttccctcgagattttattaacctttgtaaaaccttaggagaagaaatctttacatatactataataggggccaaggaggttttactgagttgagctggatgattaattgtatccgcgtcaaggaccaccaactgcaatgttcttgcaagttcaaaaatcctttcgatttcactctgaacttccgctaagcttgaccttgtgttggatctttctattattgcgtgcttactgggattgtttaataccgagcgtttggcaagcgagatgtcagcggtgacccttgtgatggatatccgcccttcaaatctgtgttttaaaaaatcaaacagcgctttttgcatcatatctgtgacctcgtagcccttcagagaagggcccactaggaccactggtcgcatggaaggtaccacatcatacggaggagtgtgctctgtcttcttaaagaagggcattcttttctctttggagtggggtgacgttacactgtttgcactgggtttaggggagcggtggtttgctggaatatcattttcttctgcatctaagccagtagcatctatgtctatagcagatgatggaggtgttgattttctggaactaggtactatgtcacccaaactggatgatgaatttcctcctgatttactggagtagaatttcccttgcttggctctctgttcatgctgcagcctcatgttttctagtttgactgggcttggaatgaatccgatttcacagccttcttttaccaatcgccctatccaccagtcattgttaaatttttccttaacatgcagaaaatcttttgcttcgaatgagatggccatgccaggcactggaacatcatcttcatgggccgcactgtagctgacatttgtccgaaccgcaaatgcaacgggctttgtctttgctttttccaactgtgcctgggcctgccgctccgcttctctgcgcactgcctcccggtcctcctccagagatacatcggaatcggatggacggctagtgtaggagtctgccgaacccccaggaataatgtatttagtttgaggagctataaggcgtctgtcaagcatgctagaccaattccaagtgcgcccagcactccagcaggaattttcttcacaggagcaagaattcaggactagctaaaaggcagccaagtcttgctttgctgaacagcatagcaactgctttcctttttcttgctggcttggggtgtgtagtcttagttagtgtgactttctaaagttcgtcggatcacaacagctctctgttccagaaccacttaggc

SEQ ID NO: 15362 - RNA, 4185 nt, Homo sapiens
  source 1..4185: mol_type = other RNA
gctgggattacaggcatgagccactgcgcccggctgatttattttgttaaataagttaatgtgcagatctgaagttaggtaattatacacaggcattttcctgggacaaacttcaagtgccaggtacttgcactcttaatactgtcttaccatccagttataactggacaaaatatacacttgagacacggaaaaggtcttagccttaaacatgatgacattgtaagcttcttacagcagtgtaattgaggcatggagataatgtcttcaaggttccccttctgtgtacatgtcttatgtaggataatattcttaacattttattcacttcaagtcaccccattttgccctgatttcttctgaagaacagaaactttggttataagaagcacttctgggttctgacagacagtgaacctgctggagtcggtggtggggaggaatggtaggtaactgggaggtaaacaaacaacaggaacaataggcaaggttagaaattgaagtgggagaagttataaaaatttattttcccacgaaataattccacaagctgtgtaaacatttcttactaaaacaaatactctaacacacaaagattgtacatttccagtgaaacactcacagtaaaattgcctgtattttcactctctaggagcaaaaacaaggaggcagcagatgaatgctttcctagttacctttggcagcaagcttactcacattccctgactgctcaatgggttgttaaagcaacatatagcacaattaattaaatacagagcgaggtgggcagaatgctcgatatcagtctctagtttcttcgttagtcttcagcattccaattcatctcaaccattcagtcactcggtgcacactttcttacatacggacacacacacgtgcatatagcgagttccggctcgtagactccagtgcagtgactagaacagacactagctactaagaatgtgtcacaatcagtgtgaactgtatggagtagaacaacctctggagttttatatttaccataatttatggtggaaattacaaacttacttacaaggatggtataacattcagaattcaaaccttttcaagtcaagcaatcacacatatttacagtatgtacacactttctactagaatgaggataggtgtctagacaatgttattacaaatttcctgaatgtgggcatttctagtccctgtaattcataaagcaaatctgctgacttggcattaagactctaaaatagtgtgatcaaactgatatatatatatattatatatataataagaaggtgtttgtttgcagaaataacatttacaaactgtctatacagtacacagtactagtacatagaaaatagattctaactttatgatcccctttgtgtaaggcaagactgaatctgtccccaaatttagtcagccagaggtacaagcaagaaacagtggtccatgaatgaatatgcaaatcagatgcctgcgtattaacgtattaaaaatctggagaaacaagaaattccactttttatctgtgctgattctggcttgttggatacatcaactacatttcttaaaacactaacatcacctgggtggcaacagattttgttcaagtggcagctacccaaaacagtttttgaagagtccagtatgcaaccggaggactgcagccataccaggccaatttatgtagcacttacaaaagaaaaagtatctcaatactctatccatgctattgctattcaagcaacagcaataatacaaaatattacaagacagatcacatatgattgcagtgtagaccccaaagactttgttttggggatgctgttagttatacaagacttcaaaaaaaaaaaaaaaaaaacacaaacgggcaaaactcattggcggatgtaaacatccctgttccactccccagcctcattccgtttttttgatatcacttctccatccttttcacagtagcgatccttggatttatgacggctgcgctgcttgttgcactcgttgtggtcctgctctcgatccacgtcccgggaacggtgccgggactccctgtgtctgtggtcactgctcccgtgggtctcgtctctgtggttgtggtcacggtgtgaggcatagtggtccacgtggtcatgggaataatcttcctttggctctacgtaggcagagtctcgactctcctgggtttccgagtcaaatgtctcttgcctggagaggccgcgacttgtcccactgcgatggttgtggtgtggggctgaggaggaagagcggtgctgggatttcttgactggttccacactaggttcttcttcagcttgggaagcagaacggataggagcggagcgatcagtcctctgatcaccttgagaaccctgtgaattagaggctagggtggggctaagaggcagacttgaagtggctaatgtacggctaaggagagggttggggaggctactgctgggaggatgggtggccttccagtaggcctccagatagtcggcaaggtgctcacaggcatcctcaagctggttctcatccaagatcacatcgaacagctctggaggacactgagccagtttatcagctgctaccatctggacgttgaggtgtttagcttgagatttccctcgagattttattaacctttgtaaaaccttaggagaagaaatctttacatatactataataggggccaaggaggttttactgagttgagctggatgattaattgtatccgcgtcaaggaccaccaactgcaatgttcttgcaagttcaaaaatcctttcgatttcactctgaacttccgctaagcttgaccttgtgttggatctttctattattgcgtgcttactgggattgtttaataccgagcgtttggcaagcgagatgtcagcggtgacccttgtgatggatatccgcccttcaaatctgtgttttaaaaaatcaaacagcgctttttgcatcatatctgtgacctcgtagcccttcagagaagggcccactaggaccactggtcgcatggaaggtaccacatcatacggaggagtgtgctctgtcttcttaaagaagggcattcttttctctttggagtggggtgacgttacactgtttgcactgggtttaggggagcggtggtttgctggaatatcattttcttctgcatctaagccagtagcatctatgtctatagcagatgatggaggtgttgattttctggaactaggtactatgtcacccaaactggatgatgaatttcctcctgatttactggagtagaatttcccttgcttggctctctgttcatgctgcagcctcatgttttctagtttgactgggcttggaatgaatccgatttcacagccttcttttaccaatcgccctatccaccagtcattgttaaatttttccttaacatgcagaaaatcttttgcttcgaatgagatggccatgccaggcactggaacatcatcttcatgggccgcactgtagctgacatttgtccgaaccgcaaatgcaacgggctttgtctttgctttttccaactgtgcctgggcctgccgctccgcttctctgcgcactgcctcccggtcctcctccagagatacatcggaatcggatggacggctagtgtaggagtctgccgaaccctggcgaacaaaactatttgaggtagtatcagatgacgtgcttccatcagatcctttaaatctgtttttccttctggctccttttccatatgactgtgcggcggctccgagcgcccccgcgggagccacgttctctagcagttccatctggatctcctgcgccaccgccgccgccgctgtgggaggcgacttggacatgtccctttggaccattggcgaaaagtcggctcggagcgaagcagccagcccccggcggcgggtcccctcctcctcgcccccgcctccccgcgctctgatcggctctgggggccgcccagggctcaggcccggccgttctcggcgcagcgccccgcagcgccccgggactcggcgccctgctgccaggcgctcagtgcgcgggacggggccggggcatcgggcgaagcgagccgctcgggaggcgggacgcgggggcgcggctgcggtgcctgggagaggggagccctcagcggggcagccggggccgggagagcgggcgcagcgcggc

SEQ ID NO: 15363 - RNA, 4544 nt, Homo sapiens
  source 1..4544: mol_type = other RNA
gctgggattacaggcatgagccactgcgcccggctgatttattttgttaaataagttaatgtgcagatctgaagttaggtaattatacacaggcattttcctgggacaaacttcaagtgccaggtacttgcactcttaatactgtcttaccatccagttataactggacaaaatatacacttgagacacggaaaaggtcttagccttaaacatgatgacattgtaagcttcttacagcagtgtaattgaggcatggagataatgtcttcaaggttccccttctgtgtacatgtcttatgtaggataatattcttaacattttattcacttcaagtcaccccattttgccctgatttcttctgaagaacagaaactttggttataagaagcacttctgggttctgacagacagtgaacctgctggagtcggtggtggggaggaatggtaggtaactgggaggtaaacaaacaacaggaacaataggcaaggttagaaattgaagtgggagaagttataaaaatttattttcccacgaaataattccacaagctgtgtaaacatttcttactaaaacaaatactctaacacacaaagattgtacatttccagtgaaacactcacagtaaaattgcctgtattttcactctctaggagcaaaaacaaggaggcagcagatgaatgctttcctagttacctttggcagcaagcttactcacattccctgactgctcaatgggttgttaaagcaacatatagcacaattaattaaatacagagcgaggtgggcagaatgctcgatatcagtctctagtttcttcgttagtcttcagcattccaattcatctcaaccattcagtcactcggtgcacactttcttacatacggacacacacacgtgcatatagcgagttccggctcgtagactccagtgcagtgactagaacagacactagctactaagaatgtgtcacaatcagtgtgaactgtatggagtagaacaacctctggagttttatatttaccataatttatggtggaaattacaaacttacttacaaggatggtataacattcagaattcaaaccttttcaagtcaagcaatcacacatatttacagtatgtacacactttctactagaatgaggataggtgtctagacaatgttattacaaatttcctgaatgtgggcatttctagtccctgtaattcataaagcaaatctgctgacttggcattaagactctaaaatagtgtgatcaaactgatatatatatatattatatatataataagaaggtgtttgtttgcagaaataacatttacaaactgtctatacagtacacagtactagtacatagaaaatagattctaactttatgatcccctttgtgtaaggcaagactgaatctgtccccaaatttagtcagccagaggtacaagcaagaaacagtggtccatgaatgaatatgcaaatcagatgcctgcgtattaacgtattaaaaatctggagaaacaagaaattccactttttatctgtgctgattctggcttgttggatacatcaactacatttcttaaaacactaacatcacctgggtggcaacagattttgttcaagtggcagctacccaaaacagtttttgaagagtccagtatgcaaccggaggactgcagccataccaggccaatttatgtagcacttacaaaagaaaaagtatctcaatactctatccatgctattgctattcaagcaacagcaataatacaaaatattacaagacagatcacatatgattgcagtgtagaccccaaagactttgttttggggatgctgttagttatacaagacttcaaaaaaaaaaaaaaaaaaacacaaacgggcaaaactcattggcggatgtaaacatccctgttccactccccagcctcattccgtttttttgatatcacttctccatccttttcacagtagcgatccttggatttatgacggctgcgctgcttgttgcactcgttgtggtcctgctctcgatccacgtcccgggaacggtgccgggactccctgtgtctgtggtcactgctcccgtgggtctcgtctctgtggttgtggtcacggtgtgaggcatagtggtccacgtggtcatgggaataatcttcctttggctctacgtaggcagagtctcgactctcctgggtttccgagtcaaatgtctcttgcctggagaggccgcgacttgtcccactgcgatggttgtggtgtggggctgaggaggaagagcggtgctgggatttcttgactggttccacactaggttcttcttcagcttgggaagcagaacggataggagcggagcgatcagtcctctgatcaccttgagaaccctgtgaattagaggctagggtggggctaagaggcagacttgaagtggctaatgtacggctaaggagagggttggggaggctactgctgggaggatgggtggccttccagtaggcctccagatagtcggcaaggtgctcacaggcatcctcaagctggttctcatccaagatcacatcgaacagctctggaggacactgagccagtttatcagctgctaccatctggacgttgaggtgtttagcttgagatttccctcgagattttattaacctttgtaaaaccttaggagaagaaatctttacatatactataataggggccaaggaggttttactgagttgagctggatgattaattgtatccgcgtcaaggaccaccaactgcaatgttcttgcaagttcaaaaatcctttcgatttcactctgaacttccgctaagcttgaccttgtgttggatctttctattattgcgtgcttactgggattgtttaataccgagcgtttggcaagcgagatgtcagcggtgacccttgtgatggatatccgcccttcaaatctgtgttttaaaaaatcaaacagcgctttttgcatcatatctgtgacctcgtagcccttcagagaagggcccactaggaccactggtcgcatggaaggtaccacatcatacggaggagtgtgctctgtcttcttaaagaagggcattcttttctctttggagtggggtgacgttacactgtttgcactgggtttaggggagcggtggtttgctggaatatcattttcttctgcatctaagccagtagcatctatgtctatagcagatgatggaggtgttgattttctggaactaggtactatgtcacccaaactggatgatgaatttcctcctgatttactggagtagaatttcccttgcttggctctctgttcatgctgcagcctcatgttttctagtttgactgggcttggaatgaatccgatttcacagccttcttttaccaatcgccctatccaccagtcattgttaaatttttccttaacatgcagaaaatcttttgcttcgaatgagatggccatgccaggcactggaacatcatcttcatgggccgcactgtagctgacatttgtccgaaccgcaaatgcaacgggctttgtctttgctttttccaactgtgcctgggcctgccgctccgcttctctgcgcactgcctcccggtcctcctccagagatacatcggaatcggatggacggctagtgtaggagtctgccgaaccctggcgaacaaaactatttgaggtagtatcagatgacgtgcttccatcagatcctttaaatctgtttttccttctggctccttttccatatgagatcttcagcaggtccagtccactcccctgattcatgtctctccatgtgcctctcccgggaaggggcgaggagggccagctggagcaacccgggagaagtctgggaggactggcaggtctcccccgcccttccccactggcttttcggaagcagagaaaaatggaagccgaggcagagccaggaaaaggcgcaaaggggcagggtccccggcgccaggagaggagcagagggtgggcaggcgacgaggggaggaggtgcgaggctagagatccctgcagtggaggcgccgggagaacccgaggtcggtgccctgcccggcggctcacaaaggaaggagaaggcgccgcgctctcgctacctgtgcggcggctccgagcgcccccgcgggagccacgttctctagcagttccatctggatctcctgcgccaccgccgccgccgctgtgggaggcgacttggacatgtccctttggaccattggcgaaaagtcggctcggagcgaagcagccagcccccggcggcgggtcccctcctcctcgcccccgcctccccgcgctctgatcggctctgggggccgcccagggctcaggcccggccgttctcggcgcagcgccccgcagcgccccgggactcggcgccctgctgccaggcgctcagtgcgcgggacggggccggggcatcgggcgaagcgagccgctcgggaggcgggacgcgggggcgcggctgcggtgcctgggagaggggagccctcagcggggcagccggggccgggagagcgggcgcagcgcggc

SEQ ID NO: 15364 - RNA, 3703 nt, Homo sapiens
  source 1..3703: mol_type = other RNA
gctgggattacaggcatgagccactgcgcccggctggaaaggttcttttaagagttccacaaagtggccaaaagtttattcttgcattttatcatgcgtatgccttggagttatgtttttggaatatgacttaagaaaacaaactttccaggtaacacgtagccggttcccatctttctagcatctctgcctttggctgatgtgacgccatacgttcctgacagttaatgttggctctgtagggatctgatgccaagtacagtcatagctcagccatgacacagggccttccagataggccagattcagtgcccttcccaacagatgcctctccatcccccacacctcccgactccaccaaaatgaagtggaagcacgtcttgagttgcccatttcttctgtgtctggtcaggcacacgtcaagaatgttggctggtgatgggctcaaggcaggcacagcccgcttcactgtgcatgtgtgcaggcttgattgacactggcaaaatctgcaaggatatttctagacattccaagtgattggttcctctgaggaaatgaaacattaaaaaaaaaaaaaaaaaaaaatatatatatatatatatatatacacatgtatatttaattatttttttaaagccacaattgaaaaaattctttgccactgggtagaattaaatctgacaggaaaccctaggagtttttattagtaccattattgttttctttggctccatgtattatgtcggtaaaatgacaaaaaaaaaaaaaggaaaaaaattgtaaaagacaaatattttgtacaaaaatacaaagttttaaaagctctttaagtatatttcatattattactaatagttggcctatatatctgtatgtctgcatatttttcctacacttgggattttagaaatgtatggcactgtttacacagtatatgcttaagttcttcccataactcaacgaccaatgataacctttttctgattggagtgttccatactttggaagacataatttgtataatcgcacggttactgacggaggagaatctatgtgattcagtccatgtgcacaatgaaaatcagcatatcaccctggggaacattttagttcccaagtctttgggtaatgacggatggtaaaaaacactagctgtcaattttttttcagtaattggttttcagtgctttttttttttcaatctgatgagaaggtgatgcaattagaaaggagtgtcctttgcctttgagagctgaaaatttgctcatgtgatcccatcacagtccgttataatgcagatgacagtactgtctccctgtctttttcgcaaatgaagttattgacgtcttcacattggaaatcgttccactgcccagcataaatcaacccagcacagtcttctcctggcccatggccatgaccccagttatccggctgtccagctttccaatttttgtagtctggagatgtcccatccagccacttccattcattttcacgctctgagtctgtgaggccgatccagtggctctctctccctaccatctgtttttttatccattgctgttcctctctagtgtttatgaaaacaagatgtgaagacttgtcttcacagaaaagctttgcatcctcaaaaatttctttctcaactgaaaaatagtagcatttgtctgtgaagttcttccagtgaggcgggcagccattgtcctccggtgctggggttggctcattctgcagggccaggggcaccaccgctcctgatgggccaggagggccgggggggcccttggggcctggcatgcctggtaccccaggcaagcctggcagtccccgaggtccaggcaccccaggctccccaacggtgccctgaagtccctggaagccaggagggccctgagggccggggagtccctctttgcctggtgggcccggggggcctgggtccccactggagccctgagggccgggcttcccaggggaaccacgggagcctttggggccctgggagcctttagatcctttgccgccacgctctccggggggaccagctggtccaattgggcctctctcacccgcagggccaggtggtccaggctcccccttctctcctttctgtcccttgttgccagttgggccagggggtccctgggatcctctgtcacctcttggacccctggggcccggtggaccttgtagtattgtaaaattcttgatgagctgaccatgcttggagtctactagcttcatttcttccataatcactgataagttggctacttcagtgtctaacctcgacctcatcaaatcttgttgcatcctgagagaaacagaatccaaacggatgttggccagggtattattcaaggaggtcagatcatctgtgtgtttggtaagggtatctgtgcaagtggtcctgacttcatttagattgctggtcagcgtccgcaggtggtgggctgtgtaactgatattgctaatgatgttcacaatatccgtctcaaagagctggaagcgttcctccagttggttgaacttgatggctgttctattctctgcatctttgtgtaagtcctgcaggtctttcaggttctgctcgttggcttgagagatagtggtgatgttctccatctgacctgtgaatgagttgagctggctgttcatatcctccagggtgtcgttgttggctttggccaacgcagagttgttggcagccagcgtctgcaagctctgcactttctccttcagccaatccgtgtccttcttggcttgaagaaaaacctgctgcagattttgaaagtcgttcttgattcgctggatagcctggcttgtgtcatccacagaccgctgcagattcgtgatgaggttcctctgctgcacctgggtcaggttcaggttgttgaggttcatgatgaccacattatgagaatacatttggttctgcagattgccctggagcacgctggtatcttgctgcagattcgtgacatagccattatacgcctggagggttttgtttacagtggtgatgaggaaagagttattctccaaagtttctttcaattgactctgcctgtccaccagagcatccccgctcgcctgtaacttctccagcgtatccttgttcttgctggttttttctgtaatctcacgaagttgctgacggagatctagaatgtctgatctgaaggtggagagttctgagttggtgctgatagctttcttcccagtttggtcacctaattttttcaggtcactttccactgctgtgagcttgtcatcataggtttggcgagatgtttccatgccacctgtgacattgtccattttctctacaactttatatcccaaaatggctactgtgattgttagcaaggcacacaaaatgtataataatatgatagaaaacttcagtgcccagttatttttacatttggtacattgtgttccttcctgaataccaaaccgcttgtaaccgaaggattgcacctcctcctcctctgcgaagtcgtctttcatggtgaccgtggggacgcaccgccggccggggagctccgcgcgagcgccgcgcagccgaggaagtcgtcccgagcggctgctcaccgcacgcccatggtagccgcgccgcgcgccggccgtctgcgcccccgtcctccctcgccgccgccggcccgcgctccccgcgctcccggctccgcgctctgct

SEQ ID NO: 15365 - RNA, 4237 nt, Homo sapiens
  source 1..4237: mol_type = other RNA
gctgggattacaggcatgagccactgcgcccgggctgagttttaattttgtgactgctctttggtagattttaaatattagaggtaggccctaaatagaaagaacaccatggtgcttttgctctcatgcatttcggttttaacgttaaagtatgaaagaaatatgagttcattttcatggataataatataactttattgtgtgcagcctttccacaccaatttagtttttctatgaaataagatttcaagtggtaaagttactgttaaggagacacactggaaaaagctgaagagtttttttgtctgaaactgaaaaacagaaaagtctagggggaaagatgtgagaaaactactataggctacaaagaccacaaaaacagttttggggattagaagggggtgacattgagtgagtgtgtgggaagagaagggctgggcaaattatctcagaagagggggtagtaggatttcaggtggatgtttaaggtatttgcttggcagatataatctaggaatctcctagctcttgcatttcctgctatctgtaactttattatgtagtataataattttttatttagcacaaagttcatttggactagagaatcggaaggtgctaattttgtccccggctagcaaagtcatacctgaggtatgcgctggaaaacaactggaagacctaggcaggggaattcaaagttgttttttttttaaattttattatcctgtcttggtttccttattgaatagatttccacaggaaaaatactgtgagtttactgatctgctgcagaattggaatttagactcacaataaagagagttaaagatagatccaaaggttcacttaaaataaaaatcaccagacagaacaggctactgaagagtctcttccccgtggttaagtttcatcatacacataaggctttggagcagctgtcctcaaatgcttctatccaaaacccactcctcttctggagtttctgaaccctttatgttccacatccacctcctctctcttcccatggctctctacagagccatttgtgacatgtctacctgacacttttggggacgtggtaagtaaaagaggcaaagtccctaacacttattagaaacgtgagaagagaaaaatgtgcttggacttgctttagtattctaattggcacacatgccaaaagactaacgatcttgtatgctgaggtggaaatgagcctctaataaaagctacgaaatcctctaatacaagatacaaaaacttatacattacaccagtctagctgaaacataattttttgatactctttgactgaactttagacagaaaagacaaaactgaaatggaggaacgtaatttaagtgtggcagaaagttgggaatcatgcggcctgatatacaaagataaatgcatcactgaggcatattcccctggccttgaggtatgcaggcaaaggagaggtcacaccttcctgggagacaaaggatcaaagttgacacagagctccaagaaaatatttaccagaagaatgtgatgattcatttatcagtccagaaatcccaagtacaaaacttcaagatacaagaaggatcaaattatatcatatatatgattcaatttaaaaattcttagccctcttatatcatattatctagattataatagtaaaaaatcaagttacattcatatgaaactttcataaaaagaaatcaaatccagttttatgaaattttatagtacaattactttctagtgggtcttttcttaggtcacagtatttataattccatttacatctttataatttttaaaattagaaaacaaaaggatgtcaatagaaatctaaattttcacttgcaaaactcccttcagtttccaggccagtaacacatggtgatgtcgacttgtcctccagacatggacggctaccaaagatccccagttcacggagcatgcaggcctctactcattaggaacgctttttggtttggctcacgtttcaagaaattgtggagcatgtccatgccgtccagagatcccccaggtttcaggattaggtttctgtatttcattccaacctctggattcattatcccttcttttttaaaacagctgtaaaacatatccatggaaaatacttcactccaaagatatccataatattggccatcgtatccccctgccaaatgtccaaaggtagctggcatatttgtgcctggagtagctgcaactcctaatatttctgagcagtatttggcatattcacttgcagcatccagcgatgtgttggtatgaagagactgatcaactttgctcaaaacaatctggcgcagggtcagaagacctgtgttgaccagcctagaagcaacaagtttttcaagcagatcgtctgcaatagggcttccatctttataatgttttgacaatcttcggagggaatcgacgtcccacacccaattttcaagcatttgcgatggcacctctacaaagtcagtttccacatttgttccgctaaatcgtgcaaaatcagtctcgtcgtgtctcaggagagagggacgacctgccactggctgtgagaagttcaccacgagggcagccactgccatcatccggcttccatcaggcagaaggcagccaggctggagaccgaagcaggccgcatgattgtattttccttcccttggatagaggtccaaatagaactgtcccaatacttctcctgtagctttatccttcacagtataaagtgtaacactcttgttccaaacatgagcatctgtcatttgttcaaatgaaagtcccaacaactcctggtaggtgttcagcaagccttcagtgaccacctcaattgggaagtattccttgaggaactcttggtctatggaatacttgagttcctctgtctgagtcatgtagtaatatagatcccaggcattgattttcccatcatattcaaaacccctgtctttgcattcctttttcttcaaattcaaaataaactctcgttctgcttcacccaagggttttaacttctggcttaaatcatctagaaaggctgttacgcggcttgtgctctttgcagtgttcatttcaaggacgaagtcagcatgtgtgctataaccgagtagtttggccaccttggttcgcagtgggagtagctgctgcaaaattatggtgttttcctctttgcaccttgtattaaaagccatttccatccttcttctggtttcagggatacaacatttcttcatgacagggaaatagtgtggatattttaaggtaattttatacttgtcatcatctgtcttttctaaactgtcaatgaaatcatcaggaagagcaccaagttcagccttggaaaatacaaggaaggtatcatcctcattgaggtttttgttaaaatcaatacatagctcactcattcttttcttcattgatttgatttcattctgtacttgttcaggaagatggagcccatttcttttccccattttaattgacttttccaagtatcgtctggcctcaggttttatcttccccagatcacaggtttcctgtaaatgaacaattctctcaaatatatctcctctcatgctcatctcaatatcaaaacgagaaagtcttttgtctgcttctgtacttgctgctcgtacttctttgtcagaggatacatgctggggaaagtctagcatggtcctttccactatatactttacttctacatctgccagtgcctgcagacagttctcgtaagttacttcctcaataccgagcattccaacagcatcgtacacctgtttggtctgcacaatgagctcctcagttcttgttttaatttgctctggtgaaagatcccatcttaaaacatttctgccagccacagtataggaagacattgcctgaagaggagacatcacttctcttcctaacgtcattctgagtaaaatcctggaaccaccaacttcaggtggctgaagcaggagaatcgcttgaaccagggaggcagaggctgcagtgagccaagatcacgccactgcacaccagcctaggcaacagagcgagactccatctgcggaggcttcgcacagccaaaaggcaccgggcgatcatgggagcgctgagaggctggcggcggcgggcgcgtggtccttcggcgtggggcggcgaggcgggcggcagcgcctgggcgcccgggagtctcgagccggcctagccgcagaggccacagtggctgcct

SEQ ID NO: 15366 - RNA, 4227 nt, Homo sapiens
  source 1..4227: mol_type = other RNA
gctgggattacaggcatgagccactgcgcccgggctgagttttaattttgtgactgctctttggtagattttaaatattagaggtaggccctaaatagaaagaacaccatggtgcttttgctctcatgcatttcggttttaacgttaaagtatgaaagaaatatgagttcattttcatggataataatataactttattgtgtgcagcctttccacaccaatttagtttttctatgaaataagatttcaagtggtaaagttactgttaaggagacacactggaaaaagctgaagagtttttttgtctgaaactgaaaaacagaaaagtctagggggaaagatgtgagaaaactactataggctacaaagaccacaaaaacagttttggggattagaagggggtgacattgagtgagtgtgtgggaagagaagggctgggcaaattatctcagaagagggggtagtaggatttcaggtggatgtttaaggtatttgcttggcagatataatctaggaatctcctagctcttgcatttcctgctatctgtaactttattatgtagtataataattttttatttagcacaaagttcatttggactagagaatcggaaggtgctaattttgtccccggctagcaaagtcatacctgaggtatgcgctggaaaacaactggaagacctaggcaggggaattcaaagttgttttttttttaaattttattatcctgtcttggtttccttattgaatagatttccacaggaaaaatactgtgagtttactgatctgctgcagaattggaatttagactcacaataaagagagttaaagatagatccaaaggttcacttaaaataaaaatcaccagacagaacaggctactgaagagtctcttccccgtggttaagtttcatcatacacataaggctttggagcagctgtcctcaaatgcttctatccaaaacccactcctcttctggagtttctgaaccctttatgttccacatccacctcctctctcttcccatggctctctacagagccatttgtgacatgtctacctgacacttttggggacgtggtaagtaaaagaggcaaagtccctaacacttattagaaacgtgagaagagaaaaatgtgcttggacttgctttagtattctaattggcacacatgccaaaagactaacgatcttgtatgctgaggtggaaatgagcctctaataaaagctacgaaatcctctaatacaagatacaaaaacttatacattacaccagtctagctgaaacataattttttgatactctttgactgaactttagacagaaaagacaaaactgaaatggaggaacgtaatttaagtgtggcagaaagttgggaatcatgcggcctgatatacaaagataaatgcatcactgaggcatattcccctggccttgaggtatgcaggcaaaggagaggtcacaccttcctgggagacaaaggatcaaagttgacacagagctccaagaaaatatttaccagaagaatgtgatgattcatttatcagtccagaaatcccaagtacaaaacttcaagatacaagaaggatcaaattatatcatatatatgattcaatttaaaaattcttagccctcttatatcatattatctagattataatagtaaaaaatcaagttacattcatatgaaactttcataaaaagaaatcaaatccagttttatgaaattttatagtacaattactttctagtgggtcttttcttaggtcacagtatttataattccatttacatctttataatttttaaaattagaaaacaaaaggatgtcaatagaaatctaaattttcacttgcaaaactcccttcagtttccaggccagtaacacatggtgatgtcgacttgtcctccagacatggacggctaccaaagatccccagttcacggagcatgcaggcctctactcattaggaacgctttttggtttggctcacgtttcaagaaattgtggagcatgtccatgccgtccagagatcccccaggtttcaggattaggtttctgtatttcattccaacctctggattcattatcccttcttttttaaaacagctgtaaaacatatccatggaaaatacttcactccaaagatatccataatattggccatcgtatccccctgccaaatgtccaaaggtagctggcatatttgtgcctggagtagctgcaactcctaatatttctgagcagtatttggcatattcacttgcagcatccagcgatgtgttggtatgaagagactgatcaactttgctcaaaacaatctggcgcagggtcagaagacctgtgttgaccagcctagaagcaacaagtttttcaagcagatcgtctgcaatagggcttccatctttataatgttttgacaatcttcggagggaatcgacgtcccacacccaattttcaagcatttgcgatggcacctctacaaagtcagtttccacatttgttccgctaaatcgtgcaaaatcagtctgtgcacaaatctgatgcatcacgtgaccaaactcatgaaagtaagtcctcacctcgtcgtgtctcaggagagagggacgacctgccactggctgtgagaagttcaccacgagggcagccactgccatcatccggcttccatcaggcagaaggcagccaggctggagaccgaagcaggccgcatgattgtattttccttcccttggatagaggtccaaatagaactgtcccaatacttctcctgtagctttatccttcacagtataaagtgtaacactcttgttccaaacatgagcatctgtcatttgttcaaatgaaagtcccaacaactcctggtaggtgttcagcaagccttcagtgaccacctcaattgggaagtattccttgaggaactcttggtctatggaatacttgagttcctctgtctgagtcatgtagtaatatagatcccaggcattgattttcccatcatattcaaaacccctgtctttgcattcctttttcttcaaattcaaaataaactctcgttctgcttcacccaagggttttaacttctggcttaaatcatctagaaaggctgttacgcggcttgtgctctttgcagtgttcatttcaaggacgaagtcagcatgtgtgctataaccgagtagtttggccaccttggttcgcagtgggagtagctgctgcaaaattatggtgttttcctctttgcaccttgtattaaaagccatttccatccttcttctggtttcagggatacaacatttcttcatgacagggaaatagtgtggatattttaaggtaattttatacttgtcatcatctgtcttttctaaactgtcaatgaaatcatcaggaagagcaccaagttcagccttggaaaatacaaggaaggtatcatcctcattgaggtttttgttaaaatcaatacatagctcactcattcttttcttcattgatttgatttcattctgtacttgttcaggaagatggagcccatttcttttccccattttaattgacttttccaagtatcgtctggcctcaggttttatcttccccagatcacaggtttcctgtaaatgaacaattctctcaaatatatctcctctcatgctcatctcaatatcaaaacgagaaagtcttttgtctgcttctgtacttgctgctcgtacttctttgtcagaggatacatgctggggaaagtctagcatggtcctttccactatatactttacttctacatctgccagtgcctgcagacagttctcgtaagttacttcctcaataccgagcattccaacagcatcgtacacctgtttggtctgcacaatgagctcctcagttcttgttttaatttgctctggtgaaagatcccatcttaaaacatttctgccagccacagtataggaagacattgcctgaagaggagacatcacttctcttcctaacgtcattctgagtaaaatcctggaaccaccaactctgcggaggcttcgcacagccaaaaggcaccgggcgatcatgggagcgctgagaggctggcggcggcgggcgcgtggtccttcggcgtggggcggcgaggcgggcggcagcgcctgggcgcccgggagtctcgagccggcctagccgcagaggccacagtggctgcctggccagcgccctcccacgtgcggcagctccacgccggcgcct

SEQ ID NO: 15367 - RNA, 2942 nt, Homo sapiens
  source 1..2942: mol_type = other RNA
gctgggattacaggcatgagccactgcgcccggttgatgcatgtgcttaagaaccactgctccagggcaggggaaactttttgtgtcaaggatcagacagtaaatattttaggctttgtatgccacataggtagggtctctgtcattcctgttgttcccttttacaactctttaaaaatgtaaaaacattcttagcttccaattgcacaaaaacaggtggcaggtggatttggccccttgagccatagcttgccaactcttgctctagggcaacacagctcccattctgggagatctggagcttcctgtggagacaggtggatttcccctttaatgagggaaataaacaacagcctccaggcatcagacaagttccccttatatagtagttgtgataccttctgacatgccaaggccaaagtaaggccagatcctgctttccattcaggcttcattaacttagtttacagtttgtgtgtatgtgtgcctgtgtgctctttcaacaaatttattcaattcacagtgatatctgttggacagagtcagcaatcctaccagacaaaactcatacacacattgattccagatgagaaacaacagtcccccaaggagcttgagaaatcacctagggcagccaagctggggaagggaagtggctgtgcattgctgtgtgtcctttaaggctctttggtcctggttgatttcctcttagaaggttccaaataaaacttccctttcctattcagtacacaccagtctttctttggtgtttaacctaatgggctgaggaagggaggcagccaggaaattatacccattaaagtgtgtggttaatgcctatatatatcatttttactcacagttagtggacttatcttttaaaacagaggtatgtggcagtggggtaagagaacttcccttattatagagaagattccaagaataggttcagacatgatttgaagaaccatgtaactctgctgccttgcacggtcccctttttagcactaataactcctaagtgtctgataatttcaaggttagcagcactcccaaagaagctgtccgggctgggtgtggtggctcatgcctgtaatcccagcaatttcagaggctgaggcgggcggatcacctgaggtcaggagttcgagaccagtctggccagcatggtgaaaccccgtctccactaaaatacaaaaattagccaggcgtggtggcaggtgccctgtaatcccagctacttgagaggctgaggcaggagaatcgcttgaatccaggaggcagagtttgcagtgagccgagatcgcgccactgcattccagcctgggcgacagagcaagactccatcttgaaaaaaaaaaaaaagaagctgcctgaccagggggcaacgaggaggaggatgtggaagggtgatgagccccaaggggacagagtcctttcccccttctttttcctgagttcagctagaattacatgggtaaaagtttccattgcttgggagaggaggaagcgaagaagaaagaggtatagaagcttccttttgatccaaggtcttttcctcaaccctggctggaaccagaatcctaaaggtttcctaacttttccaaatgatttgcttggatgtctcctccctgagagggcctcagcttctggtctccaggggacaggggttgaggaagcagctagaagacattggcctttgctaccctttttcacttttttcccctgaggtccaatcaaccagtaccagggtgtaagtatgaggcattcattgtcccaccccccaatctaccctggccttcaggccttgttggcaaaggggaaggaggacacaagtgtgcacgtagctaaggaggagctggtgaatatgggaatagactggtccttgctgaagtggggcatttagagacccttattgaagtagacataaggctcaagttctccatacttggccttgatagtgtcttggagcttcggttccagataggaaactggcaattcacatttctgtgggaaaagcccacacgccactggcaccatgaagatgaggaagcacccgctcagcatgacctgcaatggggcgtgcaggaccttgactttctgcatgaagtgcaatttctcaagcctttccatgatgactggcagcaagatcatcccaggagctgacatggtgatccgagaaataactacttgggtgatgcctatggccgcagctctccgggaatgaccaatctcattttcattcctgtccttcacgcagattccctttatgagctcctgctgtcgcatcatggggatattgacacagttagccgcagccacagcggcaaagggcacccagcggcccaccaagggcggcgctttctttgtcaacatgttcatgcccacagccgtggccacagcagtggttgtggctgtgaagtaggaaagggccatctgcctgactgatgtgggggaagccgcattcctgttggtgtagttgactaaggcattgaaggactggttcacccactgccagaagatcaccgccggcatcgtcctgtagaactggagcatgaagcccgtgatgatcatgccgccaggaagctggaaagacatgcgcccgatgacattcatcttctccccagtgtcggggtggaaggccgagtcatacagcttcttggcatacagcagctgctccacttgggtgcctgggggcacaacccccatcctgctcttctccaccatcaccttggcccagtccagctcccgctcagatacaaagacagtgcgggggtccgtgatgtttaggaagtgcttcactctccccaggaaggtgcgctggtcccaacggggggcatcgatgttaaagccagacaggtcagcctccatcttgctcacacataaaactgtggacctggtcccgggacaaatgccaccagttacagcccgccttgaaaact

SEQ ID NO: 15368 - RNA, 3040 nt, Homo sapiens
  source 1..3040: mol_type = other RNA
gctgggattacaggcatgagccactgcgcccggttgatgcatgtgcttaagaaccactgctccagggcaggggaaactttttgtgtcaaggatcagacagtaaatattttaggctttgtatgccacataggtagggtctctgtcattcctgttgttcccttttacaactctttaaaaatgtaaaaacattcttagcttccaattgcacaaaaacaggtggcaggtggatttggccccttgagccatagcttgccaactcttgctctagggcaacacagctcccattctgggagatctggagcttcctgtggagacaggtggatttcccctttaatgagggaaataaacaacagcctccaggcatcagacaagttccccttatatagtagttgtgataccttctgacatgccaaggccaaagtaaggccagatcctgctttccattcaggcttcattaacttagtttacagtttgtgtgtatgtgtgcctgtgtgctctttcaacaaatttattcaattcacagtgatatctgttggacagagtcagcaatcctaccagacaaaactcatacacacattgattccagatgagaaacaacagtcccccaaggagcttgagaaatcacctagggcagccaagctggggaagggaagtggctgtgcattgctgtgtgtcctttaaggctctttggtcctggttgatttcctcttagaaggttccaaataaaacttccctttcctattcagtacacaccagtctttctttggtgtttaacctaatgggctgaggaagggaggcagccaggaaattatacccattaaagtgtgtggttaatgcctatatatatcatttttactcacagttagtggacttatcttttaaaacagaggtatgtggcagtggggtaagagaacttcccttattatagagaagattccaagaataggttcagacatgatttgaagaaccatgtaactctgctgccttgcacggtcccctttttagcactaataactcctaagtgtctgataatttcaaggttagcagcactcccaaagaagctgtccgggctgggtgtggtggctcatgcctgtaatcccagcaatttcagaggctgaggcgggcggatcacctgaggtcaggagttcgagaccagtctggccagcatggtgaaaccccgtctccactaaaatacaaaaattagccaggcgtggtggcaggtgccctgtaatcccagctacttgagaggctgaggcaggagaatcgcttgaatccaggaggcagagtttgcagtgagccgagatcgcgccactgcattccagcctgggcgacagagcaagactccatcttgaaaaaaaaaaaaaagaagctgcctgaccagggggcaacgaggaggaggatgtggaagggtgatgagccccaaggggacagagtcctttcccccttctttttcctgagttcagctagaattacatgggtaaaagtttccattgcttgggagaggaggaagcgaagaagaaagaggtatagaagcttccttttgatccaaggtcttttcctcaaccctggctggaaccagaatcctaaaggtttcctaacttttccaaatgatttgcttggatgtctcctccctgagagggcctcagcttctggtctccaggggacaggggttgaggaagcagctagaagacattggcctttgctaccctttttcacttttttcccctgaggtccaatcaaccagtaccagggtgtaagtatgaggcattcattgtcccaccccccaatctaccctggccttcaggccttgttggcaaaggggaaggaggacacaagtgtgcacgtagctaaggaggagctggtgaatatgggaatagactggtccttgctgaagtggggcatttagagacccttattgaagtagacataaggctcaagttctccatacttggccttgatagtgtcttggagcttcggttccagataggaaactggcaattcacatttctgtgggaaaagcccacacgccactggcaccatgaagatgaggaagcacccgctcagcatgacctgcaatggggcgtgcaggaccttgactttctgcatgaagtgcaatttctcaagcctttccatgatgactggcagcaagatcatcccaggagctgacatggtgatccgagaaataactacttgggtgatgcctatggccgcagctctccgggaatgaccaatctcattttcattcctgtccttcacgcagattccctttatgagctcctgctgtcgcatcatggggatattgacacagttagccgcagccacagcggcaaagggcacccagcggcccaccaagggcggcgctttctttgtcaacatgttcatgcccacagccgtggccacagcagtggttgtggctgtgaagtaggaaagggccatctgcctgactgatgtgggggaagccgcattcctgttggtgtagttgactaaggcattgaaggactggttcacccactgccagaagatcaccgccggcatcgtcctgtagaactggagcatgaagcccgtgatgatcatgccgccaggaagctggaaagacatgcgcccgatgacattcatcttctccccagtgtcggggtggaaggccgagtcatacagcttcttggcatacagcagctgctccacttgggtgcctgggggcacaacccccatcctgctcttctccaccatcaccttggcccagtccagctcccgctcagatacaaagacagtgcgggggtccgtgatgtttaggaagtgcttcactctccccaggaaggtgcgctggtcccaacggggggcatcgatgttaaagccagacaggtcagcctccatcttgctcacacataaaactgtggacctgtaatcccagctacttgggaggctaaggcaggagaatcgtttgaacccgagaggtggaggttgtgatgagccgagatcgcaccgttgcactccagcctggtcccgggacaaatgccaccagttacagcccgccttgaaaact

SEQ ID NO: 15369 - RNA, 2799 nt, Homo sapiens
  source 1..2799: mol_type = other RNA
gctgggattacaggcatgagccactgcgcccggttgatgcatgtgcttaagaaccactgctccagggcaggggaaactttttgtgtcaaggatcagacagtaaatattttaggctttgtatgccacataggtagggtctctgtcattcctgttgttcccttttacaactctttaaaaatgtaaaaacattcttagcttccaattgcacaaaaacaggtggcaggtggatttggccccttgagccatagcttgccaactcttgctctagggcaacacagctcccattctgggagatctggagcttcctgtggagacaggtggatttcccctttaatgagggaaataaacaacagcctccaggcatcagacaagttccccttatatagtagttgtgataccttctgacatgccaaggccaaagtaaggccagatcctgctttccattcaggcttcattaacttagtttacagtttgtgtgtatgtgtgcctgtgtgctctttcaacaaatttattcaattcacagtgatatctgttggacagagtcagcaatcctaccagacaaaactcatacacacattgattccagatgagaaacaacagtcccccaaggagcttgagaaatcacctagggcagccaagctggggaagggaagtggctgtgcattgctgtgtgtcctttaaggctctttggtcctggttgatttcctcttagaaggttccaaataaaacttccctttcctattcagtacacaccagtctttctttggtgtttaacctaatgggctgaggaagggaggcagccaggaaattatacccattaaagtgtgtggttaatgcctatatatatcatttttactcacagttagtggacttatcttttaaaacagaggtatgtggcagtggggtaagagaacttcccttattatagagaagattccaagaataggttcagacatgatttgaagaaccatgtaactctgctgccttgcacggtcccctttttagcactaataactcctaagtgtctgataatttcaaggttagcagcactcccaaagaagctgtccgggctgggtgtggtggctcatgcctgtaatcccagcaatttcagaggctgaggcgggcggatcacctgaggtcaggagttcgagaccagtctggccagcatggtgaaaccccgtctccactaaaatacaaaaattagccaggcgtggtggcaggtgccctgtaatcccagctacttgagaggctgaggcaggagaatcgcttgaatccaggaggcagagtttgcagtgagccgagatcgcgccactgcattccagcctgggcgacagagcaagactccatcttgaaaaaaaaaaaaaagaagctgcctgaccagggggcaacgaggaggaggatgtggaagggtgatgagccccaaggggacagagtcctttcccccttctttttcctgagttcagctagaattacatgggtaaaagtttccattgcttgggagaggaggaagcgaagaagaaagaggtatagaagcttccttttgatccaaggtcttttcctcaaccctggctggaaccagaatcctaaaggtttcctaacttttccaaatgatttgcttggatgtctcctccctgagagggcctcagcttctggtctccaggggacaggggttgaggaagcagctagaagacattggcctttgctaccctttttcacttttttcccctgaggtccaatcaaccagtaccagggtgtaagtatgaggcattcattgtcccaccccccaatctaccctggccttcaggccttgttggcaaaggggaaggaggacacaagtgtgcacgtagctaaggaggagctggtgaatatgggaatagactggtccttgctgaagtggggcatttagagacccttattgaagtagacataaggctcaagttctccatacttggccttgatagtgtcttggagcttcggttccagataggaaactggcaattcacatttctgtgggaaaagcccacacgccactggcaccatgaagatgaggaagcacccgctcagcatgacctgcaatggggcgtgcaggaccttgactttctgcatgaagtgcaatttctcaagcctttccatgatgactggcagcaagatgctgtcgcatcatggggatattgacacagttagccgcagccacagcggcaaagggcacccagcggcccaccaagggcggcgctttctgactgatgtgggggaagccgcattcctgttggtgtagttgactaaggcattgaaggactggttcacccactgccagaagatcaccgccggcatcgtcctgtagaactggagcatgaagcccgtgatgatcatgccgccaggaagctggaaagacatgcgcccgatgacattcatcttctccccagtgtcggggtggaaggccgagtcatacagcttcttggcatacagcagctgctccacttgggtgcctgggggcacaacccccatcctgctcttctccaccatcaccttggcccagtccagctcccgctcagatacaaagacagtgcgggggtccgtgatgtttaggaagtgcttcactctccccaggaaggtgcgctggtcccaacggggggcatcgatgttaaagccagacaggtcagcctccatcttgctcacacataaaactgtggacccctcagttcctctcacagggtacatcatgtccagctttcagtgaaaaattacaaggcatactggtcccgggacaaatgccaccagttacagcccgccttgaaaact

SEQ ID NO: 15370 - RNA, 2576 nt, Homo sapiens
  source 1..2576: mol_type = other RNA
gctgggattacaggcatgagccactgcgccgggcctaaagtcatattttttatttagtatatttggatataatattgaaatatctttgaaggttataggactctagattaaggttcaaaaaatatttttccattcttaataatgtgcctttaaatagcagtttttaaaatccagaatatattttttaaaactagttaaaaatatttgttataaacaaatctgttattctaaacactagcatgctaagtacctttacttcataaatatatgctattttctagtttttatgtttaaaaaccagtcatcttttatttgaaaaattaagaaaaatataaaatactatacaatttttagtcacttggggtattaaagtcagaagtaaaaatctatcctccttctgtctaattctactttacaggtaactattctttaaagactgatgctttatctctagattacttctatgcttatgcaaatatatttatagctatgtatcttcatctatttacctctccattacacacatgtgtataggtatattcacattttaataatggatcaatgatatagctacacatatgtatgatatacatgcatatatttaatctcctttttgctttaaaatatgattgacatgtttccatgtcaatatatattgttaatctttgatccatttaaaattataaaatgttttcataagcaatacatccacctctgttaatttaacatatgaaagcatctatctcattgcagtgtgatttccttcaatgcagtgaactctgtggtttctccatttcttagagtatagcatagtgcacactgtctaacacatggcgggatgtcaaaacatatattgatggtaagatgaatgactgaatataaaggaagaatatcaacattaatttagtgaagcatttcctgtctgcttgctgcagtacttcacttttcaaacaaccaagcatacccctacctccaggctgcatgcatactcttccctttgcttggtgtgtctttccctcagatgtccacttgaattactccttcaccctgttgatataccattccctttctgaggactttcctgatcctaaatgtaaaatggcatcctttgtctcttcatcactgtattttactaaatctttttcatatacaaatgttttctctctatttatgtacttgcttaatgcctgtctcctccactacccctcatgagagctggacttgtcatttcccctcactgctgtacttcctgtgcctgaaacactggctgacataagatacatgcttgttcaatactggttgagtgaataagtaaatgataaaattcgatgacttccatttgtaactctctctatataattagcgagatggtgattgttaactcaagtcagaaaactcagctcctgtttgacacatgtaacatgaggcagtcattttcttacctttaacttttttattttagttgcagctaaagcatttattggtataacaaacacaaggactgccacccctgctaacactgctggacccagctcttgccaaaggagatatacggccattaggatttgaaaaggggcagaccagaggagattgaggtttgctgtcaagtccatgagttgctgacatcaagttaataatttccccagtggaaaacttttgtcgagaaacatttgataaaagtaaggcctttttgtagatcagtccatttacagctgtcttaacttttgctgaggtgagcatgttaaaacgttgatattgctgaagaatcagagtttgcaaaaagactacaacaagaagtgccactgcatagccatagccattccagccaaaatctgagctgtgttcacagaaaatgataatttgcttcattatgagtgggctagtgaaggacaaaatatcagcaaacactttgaataaggcaacttgaatcaggatggatttaaaggtgttccacaatgcatagagtagagatggtttcttgatatgtgcctctttataacaagatacctttactttttgcctctcttgattccttaaaacttcctttctccattgtttttcaaagatgggacacgcagtgcagaaggaatcactttcctttagttcaaaaagatcctctctttccaaaggtctcttatagcctaaagtaattactctgctaaaccaggaatatgtcactttactgaaaaatgaggcacttttctctggactgcatttctgtgtatcaagcgccccgcggacccgctgataggagccgcccgcgttctgcgtactggagagcatggtccgcggggcgcctggccgctggctgagagcccggctgcggctgtcacttcccttggcagcggacagtcagttcagcgccagcacggtgggaggacacgcactccgccccggcagagtcagctgtcaccttagtccctgcctttcagtcctacccagtgcgcctggggcggtgcgggcagtcagctttcaccttagtccttgccttccagtcctagccagtgcgcctggggcggggtgctggtggaatggggttgggcctggaggaggcaaggtgtggagggagacgggaa

SEQ ID NO: 15371 - RNA, 2530 nt, Homo sapiens
  source 1..2530: mol_type = other RNA
gctgggattacaggcatgagccactgcgcctgaccaacttttcccagtttctcaatgaagccataaactttcagatctcattggttgtgagagtgagaattcgatccaagtcttctaccaactgcttgaacgttggtctctgggagggcactgcatgccaacagtccctcatcatcatgtacagttcgttggtgcagttggctggcttatccattctgtgtccttccttcagcagcttaaaaagttcctccacgggaatccctgggtagggcgagccccctaaagtgaagatctcccacattaacaccccgaaggaccagacatcactctgatgagtgtatactctatcaaacagggcttctggagccatccacttgactggaagccgcccattggtggtctttttgtaatagtctatattgttgatatctctggcgagtccaaagtctgctattttcatcacattgttttctgttaccaaaacatttctggctgctaaatctcgatgaatacatttttgggaagccaagtactccatgcctctggccagctggtaggtgcatgacaccaagtccttgaaggtcatctgctcctcaggaacacggttaatgtcataggagtactccatcccgggtggcctccgggctcggaggtattctcggaggttgcctttagaggcatactcaactatgacatagagaggcccatcctgtgtgcaggctccaagaagatttatgatattcttgtgtttcccaatcatcttcatcatctccatctctgacaccagatcagaaaggtctttctctgtggcatcatctttcaacatcttcacggccacggtgaccgcctccttgggcttgtctttgtcaattcccactgcttccgccatgaccacttgcccaaagcaaccttctcccaggggcttgcccagtgtcagcttatctcttggaaactcccattttgggtcctctggaagttcatactcggagacccctgccagcatgggggtgtctgccgttgaagagaggcgtgttgttatcctcaccagcggggtgttggagttcatggaggagctggactcagccgaaactgttacctgtctccgcagggggatacgtttggtcagcttgtgcacagccggctggctgctgaagtctggcttcttggtcgtgttcttcattcggcacaggatgactgttaccaccatacaggcgattaagaagacccctatgcagtaaatggctatctccaggtagtctggggaagctgtaatctccttttctcttccaggcgcttgctgttttggcaggacagtgagccaggcagactggttggcctgccctatataattggagaccttacatatatattccccagcatccgcctcggtcacattgaacagagccagcacttctgcattggaactatttatccccgagtgcttgagaaccttgaggtagggcagcccgtcgggcccgtatttactgccgttcttttccacgtgcttgatccactggatgtggggctgggcatcactgtaaaccttgcagacaaactctacgtctcctccgaccactgtggaggcatttgccggcagtccggcttggaggatgggccggtgaggcgatcgctccacaacatccaggtggtacgtgtgattgatggacccgtattcattctccactacacaggtataatttcccttgtcagatgggaccacactttccataatgaggctccagtgctggtttcgtaccttgtagcctccaatgcgatgctcctgcttaaactccttcccgtttttcagccaccgcatggttggcattgggttccccccggctgggcagcgaaacttgacagtgttggccgcaggcacagcatggagccgcttttccatcttttctgtgttggtccagtatggtgctctcttgttgttactgttctcactgacaaaatcttccgcaccatcggtgtcatcctcatcatctccggatgagatggcatctgtgacattcaccatgaagtaccaagtttcactgtctacagtcctactggcagtacaagcatagaggccggagtctctaggcgtggcgccctttatctgcaagtactccccaataagcactgtcctattgttgggccccaagtgcaccccatccttagtccaactgatcacggcggcatctttcaacaggcagcgcacctctagcgactcccctggcgcagccacgtacacttctggttgagagatttggtatttggttggtggctcttctggctctaatgtggtatcctcaactaaactgaaggagggccgggccagggacaaggttgccatggtgaccacgaccaggcagatgaaacgaccccagctgaccatggttacggtaccaatccccggtcctcttccatatctccatgtggacgttaatcccatctgcacacttcctctacgggcatggactacgcgcaatgccttcagcctgcggtgggctcaggaaccgaggcgctgccgctgctgctgcagtca

SEQ ID NO: 15372 - RNA, 2746 nt, Homo sapiens
  source 1..2746: mol_type = other RNA
gctgggattacaggcatgagccactgcgcctgaccaacttttcccagtttctcaatgaagccataaactttcagatctcattggttgtgagagtgagaattcgatccaagtcttctaccaactgcttgaacgttggtctctgggagggcactgcatgccaacagtccctcatcatcatgtacagttcgttggtgcagttggctggcttatccattctgtgtccttccttcagcagcttaaaaagttcctccacgggaatccctgggtagggcgagccccctaaagtgaagatctcccacattaacaccccgaaggaccagacatcactctgatgagtgtatactctatcaaacagggcttctggagccatccacttgactggaagccgcccattggtggtctttttgtaatagtctatattgttgatatctctggcgagtccaaagtctgctattttcatcacattgttttctgttaccaaaacatttctggctgctaaatctcgatgaatacatttttgggaagccaagtactccatgcctctggccagctggtaggtgcatgacaccaagtccttgaaggtcatctgctcctcaggaacacggttaatgtcataggagtactccatcccgggtggcctccgggctcggaggtattctcggaggttgcctttagaggcatactcaactatgacatagagaggcccatcctgtgtgcaggctccaagaagatttatgatattcttgtgtttcccaatcatcttcatcatctccatctctgacaccagatcagaaaggtctttctctgtggcatcatctttcaacatcttcacggccacggtgaccgcctccttgggcttgtctttgtcaattcccactgcttccgccatgaccacttgcccaaagcaaccttctcccaggggcttgcccagtgtcagcttatctcttggaaactcccattttgggtcctctggaagttcatactcggagacccctgccagcatgggggtgtctgccgttgaagagaggcgtgttgttatcctcaccagcggggtgttggagttcatggaggagctggactcagccgaaactgttacctgtctccgcagggggatacgtttggtcagcttgtgcacagccggctggctgctgaagtctggcttcttggtcgtgttcttcattcggcacaggatgactgttaccaccatacaggcgattaagaagacccctatgcagtaaatggctatctccaggtagtctggggaagctgtaatctccttttctcttccaggcgcttgctgttttggcaggacagtgagccaggcagactggttggcctgccctatataattggagaccttacatatatattccccagcatccgcctcggtcacattgaacagagccagcacttctgcattggaactatttatccccgagtgcttgagaaccttgaggtagggcagcccgtcgggcccgtatttactgccgttcttttccacgtgcttgatccactggatgtggggctgggcatcactgtaaaccttgcagacaaactctacgtctcctccgaccactgtggaggcatttgccggcagtccggcttggaggatgggccggtgaggcgatcgctccacaacatccaggtggtacgtgtgattgatggacccgtattcattctccactacacaggtataatttcccttgtcagatgggaccacactttccataatgaggctccagtgctggtttcgtaccttgtagcctccaatgcgatgctcctgcttaaactccttcccgtttttcagccaccgcatggttggcattgggttccccccggctgggcagcgaaacttgacagtgttggccgcaggcacagcatggagccgcttttccatcttttctgtgttggtccagtatggtgctctcttgttgttactgttctcactgacaaaatcttccgcaccatcggtgtcatcctcatcatctccggatgagatggcatcttctggctctaatgtggtatcctcaactaaactgaaggagggccgggccagggacaaggttgccatggtgaccacgaccaggcagatgaaacgaccccagctgaccatggttacggtaccaatccccggtcctcttccatatctccatgtggacgttaatcccatctgcacacttcctctacgggcatggactacgcgcaatgccttcagcctgcggtgggctcaggaaccgaggcgctgccgctgctgctgcagtcacttgaatggcaacgctcctccgcgacctgtgttgtccccgcgccccgcgtgggtcgggatggagaaagcgacgagcccggggttgcggggagcaactccaaacgcagaagagtggtccttgggtcttcgccggcgccaagcctcccgggcttcacgcgtaccccaggctgcggaggagcgcgggcatgacgcccgcgggctgccctcggatttggggaacgagaggaagaaaggactcaggcttggcgttgcctccaccaaactttgctcgcgagttgcgaaggctcagagcgcgcaggcaagctgcggcctcggggcccccggggctcgcggccggcccccgccagcccggagagcagtcgccgcgccgggccaggtacgccgcatgcagccccgcggcgcccgagctttgtggcggccgcgcgcgctccctcgcccgctccgcacccgccgcccgcccgctcggctctccaccgcgctctc

SEQ ID NO: 15373 - RNA, 954 nt, Homo sapiens
  source 1..954: mol_type = other RNA
gctgggattacaggcatgagccactgcgcctgacctactcaagagttttcttagggctcccttaatgtctttatttctcagactgtaaatgaatgggttcaacatgggagtgactgctgtgtatatcactgaagcaattatgttcttgtcattggtgttgctggatgggggaagaaaatagagaccaataattgtccgataatagatagtcaccactgagaggtgggatccacaagtggacaaggctttgcatatgcccttggtagagggaatctggaggatggtgaccccaatgtgaccataagaaaccaggatgcacaggaatggaagcataatggctgtcaatgctgctgtaaagattgctaactgattgagggaggtgtctgagcaggacaacttgagcagggcaccaaggtcacagaagtagtgagggatgatgtggtcagcacagaaggaaagctgggccaggaggagggtatgcaaaagagcacacgcacaagcgatgacccaggacccagccaccagcatgacacactggctctgagtcatgatggtggcataatgtagaggatgacagatggccacatacctgtcatatgccattgaagtgataaggaaactgtctaagtcagcaaaaaatatgaaaaaatatgtctgtgaaatgcatcccttgtaaaagacggctaggtgctgagtctgcatgttcatcagcatcttagggacagtgacagatgaaaaggagatgtcagtgagggccaagtggctaaggaagaagtacatgggggtgtgaaggtgagagtctagctggatgagcagcatgatgagcaggttccccagcaccgtggtcaggtacatgcccaggaacagggcgaagaacacggcctgctgctctggccggatggggaggcccaggaggaggaactcggacacgctgctctggttctcagggctcat

SEQ ID NO: 15374 - RNA, 733 nt, Homo sapiens
  source 1..733: mol_type = other RNA
gctgggattacaggcatgagccactgcgcctggactaattttttattttttgtagagacagagtttctctgtgttgcctaggctggtctcaaactcctggtctgaagagatcctcaggcctcagcctcccaaagtgctgggactacaggcataagccatcatgtcccactgcatttccaattattaacaattattttcacttacaataaatgaattggatggtgccaatctccattttctagaccttacattctctttcagctactgctcagctttctccatctctcctttcttcttgaggcagtcttctattttgtacattatacattcctgggtccatgggaatagagctgtggttgttcaacgctgtagctccctcctcatcttcatcttcactctctaatggtgggtctggcaaatgaagccccagggcctggattcgatcctggatgtcagcaactacatctccatcccccactggtgccagttccacctcctcttgttcaggatcttggttcaggggctggtaggagtagccagctgggcccgaccccgtttcctcctgctcttcctcaggctcctcactgctccaatccccagtgccttctgaagggccctgatgtcccagttcctcagtctgattggggaagatacgctcagggcccatggtgtctcctcctagaactactgttgccatccgggcaggggccgctcagagcccgcggcctccact

SEQ ID NO: 15375 - RNA, 3348 nt, Homo sapiens
  source 1..3348: mol_type = other RNA
gctgggattacaggcatgagccactgcgcctggcatgacaagtgattttcatactaaagttaattaaaatagacccaagaatcatatacaaacagggggaagagaggataaaaatgaccaagagcaactgaagccattcttgttgcaacttcctttccaaaggaaagcagaggcactgggagtgcagagatggcctcccgactccttgtcccagtgagaggcctgttgcgagccctgaccctttctcatcccaaaggcaaagctgaatctgggatgaggacaaggtacgtcctctggacctaggctatccccctaccctgtctctggctccaagtgggaagccagtcctgccctggcccagtgcagctgccaaggggacaaaaacagacccccagacacctttcagcttcgggtgaatcactttaatgctgttaacggcaagtctgtaaaaggttcaggacaaagttcttttttctttcttttttaattataaaactaacagctgttagaatctttttttctttttttccttttttcttttcccagctacaaaatactctggggagatgcattataatttaaaatatataatattgcacaaacaaccaaaaggttaattaaactaaagaaataattacaaagagaaaaaccccatcccgtcaaaaaaaagattcagcattctctccatcccaccccctcactgaaggtttgaagtggaagtgacctcactctctcggtgtccctgacccacgatccctttcactcattggtgagcacaccagattaggtacaagaatcaccagagcagcatcgtgaagcaccaggctctccagagattcctgcagcccctcattcccccagaggtgcagctttaccagagtggagggtgagagcacaaaggctgggtctgtcttcaggaagaagagcttttgcagaagcctgatgagagtttcaagttcacccccaggatagcccttccagaagcagaagggctgaggcggagaagctaggcttaccagagttgtaagtactcggctttgatcaccgctctgtaccgctggtagctgttttgtgtcctaaactacaggggagttgaggtgggtagctggttggacaaggtatcctgccaggcaacacacagaagggcctgaagtagccccctcccttcttggggaggggaagaaacgcaagagcgaactcctgcaggtggcacagctgggctaaggacttgggtgcatccgacatgaagaagccctgggaaggcatggggacagaccagcgtgggctggaggaaaggaaggaggtgggtcagggtttggtctctggattctgaaccccaaaggagcctttccaggaatggaaaatgcctgggagggggagagtcccaagagaggcaaatttcccagagataagtgcctcttacccactgggataggaaccaaaatgtgttcactgtccctgtttagccaagggtaggtggcatggccctccctgcctgcttatgtatggacagagtatgttgtctcagcttcctccgagagagactggtggtttagcttctgtctacacaggcagaagggctagaactatcccttgggacttcccagcaggagtcctcaggaacagtgggtgttcagcagaaaaacacaggctcttctggtgaggaggataggtttcctctcccttgggtcatcctattgttggcacaagtcagagtttctggccgggatttagagagccccttcccaggtgtgagcagaggcccaagagggccagcagggagccaccagaatctgtgcccagagctctggttggcagaggagatttgggggaacattctcagtcttccagggctgggctgagacgagcgagggaggcgagagatgccatgggtgggggagctgctccctctggctccctcactcccagtcctcccactctacatcttccagctccccggaggcatccactttggaaagtgccatctgcacctcctcttcagtcatgtccaagtcaaagtctttctcccagtcctcactgatgtccgtgcttgagcctcggaaaaggcaggttactaaagagcggagaagcactttggcccagaggctccaagagagtcacagaaatcttccagaggaaatcaacagtgaactgagaccttgtctctttctttccattgttggagggtgtagacttcccactatccgagttcagctcaaacacccgtaagtctgtgggcgcctcctccctcagagtctctactctggctggaggcctgggctctgggccgccggtgtggccagcaggcgttaggggcttggagtgaatagggggtgagggtccagtctcacccacatccacagccaggccctgttcctccaaggatgcctctagcagcttttgggacaggtccttgggtagcactcgtgcctcaggtgcagtggccgggttggcgatctgtgtcacgagggagatgctctcactgctctctgatggagtcacctctgctgggggctcaactgaagtcaccagattctcttcacaggggctctgggggccaggttctccttcagggaatgtagaaattttggccacaggaacctttgcctcttttggagatatgggtgaaatgcccatgagctcctcttcctcctcctcccagccgggctcttcagagatgctctgttccgcccgctgcttcagggcgtccctccgggcctgctcctgctctaactgatggactttatagaaataccgatgccagaattctgaatgggaaacagctgctggaaccatcttggtgtagagggcccggatggaggggctgcctacaaggagctctgagatctcccccttcttctcctccaagcagaactgggaaagccaggcgtcaaacaattccgggggcccatctggttcattacagtaggttgctgggtccgactgcaggctatagaggcgagccttggtgccatcatagggctcagctgtgccagacggtgtgcccatcagggtgatgacatcgcagtcgatggttttgtctggcgaaggggcaaaggtgtctgagatcacccctaggaagtcagataaccctttcttcatcttctctgttgctcctgaggagccttccgtagccagcttctccttgaccacgctggccgtggctgcgatggtacaggccgtgtcatgctgcaccacctgggtaaactccgtcaggtcccgcttcataaactccaaggcttcagaggacttctctttgactgcttggtagctctgctgcagccagctccgccaccatcccacgtcctccccttccgccatcttgcctgcatgacatcaccactattt

SEQ ID NO: 15376 - RNA, 3071 nt, Homo sapiens
  source 1..3071: mol_type = other RNA
gctgggattacaggcatgagccactgcgcctggcatgacaagtgattttcatactaaagttaattaaaatagacccaagaatcatatacaaacagggggaagagaggataaaaatgaccaagagcaactgaagccattcttgttgcaacttcctttccaaaggaaagcagaggcactgggagtgcagagatggcctcccgactccttgtcccagtgagaggcctgttgcgagccctgaccctttctcatcccaaaggcaaagctgaatctgggatgaggacaaggtacgtcctctggacctaggctatccccctaccctgtctctggctccaagtgggaagccagtcctgccctggcccagtgcagctgccaaggggacaaaaacagacccccagacacctttcagcttcgggtgaatcactttaatgctgttaacggcaagtctgtaaaaggttcaggacaaagttcttttttctttcttttttaattataaaactaacagctgttagaatctttttttctttttttccttttttcttttcccagctacaaaatactctggggagatgcattataatttaaaatatataatattgcacaaacaaccaaaaggttaattaaactaaagaaataattacaaagagaaaaaccccatcccgtcaaaaaaaagattcagcattctctccatcccaccccctcactgaaggtttgaagtggaagtgacctcactctctcggtgtccctgacccacgatccctttcactcattggtgagcacaccagattaggtacaagaatcaccagagcagcatcgtgaagcaccaggctctccagagattcctgcagcccctcattcccccagaggtgcagctttaccagagtggagggtgagagcacaaaggctgggtctgtcttcaggaagaagagcttttgcagaagcctgatgagagtttcaagttcacccccaggatagcccttccagaagcagaagggctgaggcggagaagctaggcttaccagagttgtaagtactcggctttgatcaccgctctgtaccgctggtagctgttttgtgtcctaaactacaggggagttgaggtgggtagctggttggacaaggtatcctgccaggcaacacacagaagggcctgaagtagccccctcccttcttggggaggggaagaaacgcaagagcgaactcctgcaggtggcacagctgggctaaggacttgggtgcatccgacatgaagaagccctgggaaggcatggggacagaccagcgtgggctggaggaaaggaaggaggtgggtcagggtttggtctctggattctgaaccccaaaggagcctttccaggaatggaaaatgcctgggagggggagagtcccaagagaggcaaatttcccagagataagtgcctcttacccactgggataggaaccaaaatgtgttcactgtccctgtttagccaagggtaggtggcatggccctccctgcctgcttatgtatggacagagtatgttgtctcagcttcctccgagagagactggtggtttagcttctgtctacacaggcagaagggctagaactatcccttgggacttcccagcaggagtcctcaggaacagtgggtgttcagcagaaaaacacaggctcttctggtgaggaggataggtttcctctcccttgggtcatcctattgttggcacaagtcagagtttctggccgggatttagagagccccttcccaggtgtgagcagaggcccaagagggccagcagggagccaccagaatctgtgcccagagctctggttggcagaggagatttgggggaacattctcagtcttccagggctgggctgagacgagcgagggaggcgagagatgccatgggtgggggagctgctccctctggctccctcactcccagtcctcccactctacatcttccagctccccggaggcatccactttggaaagtgccatctgcacctcctcttcagtcatgtccaagtcaaagtctttctcccagtcctcactgatgtccgtgcttgagcctttctttccattgttggagggtgtagacttcccactatccgagttcagctcaaacacccgtaagtctgtgggcgcctcctccctcagagtctctactctggctggaggcctgggctctgggccgccggtgtggccagcaggcgttaggggcttggagtgaatagggggtgagggtccagtctcacccacatccacagccaggccctgttcctccaaggatgcctctagcagcttttgggacaggtccttgggtagcactcgtgcctcaggtgcagtggccgggttggcgatctgtgtcacgagggagatgctctcactgctctctgatggagtcacctctgctgggggctcaactgaagtcaccagattctcttcacaggggctctgggggccaggttctccttcagggaatgtagaaattttggccacaggaacctttgcctcttttggagatatgggtgaaatgcccatgagctcctcttcctcctcctcccagccgggctcttcagagatgctctgttccgcccgctgcttcagggcgtccctccgggcctgctcctgctctaactgatggactttatagaaataccgatgccagaattctgaatgggaaacagctgctggaaccatcttggtgtagagggcccggatggaggggctgcctacaaggagctctgagatctcccccttcttctcctccaagcagaactgggaaagccaggcgtcaaacaattccgggggcccatctggttcattacagtaggttgctgggtccgactgcaggctatagaggcgagcagccagcttctccttgaccacgctggccgtggctgcgatggtacaggccgtgtcatgctgcaccacctgggtaaactccgtcaggtcccgcttcataaactccaaggcttcagaggacttctctttgactgcttggtagctctgctgcagccagctccgccaccatcccacgtcctccccttccgccatcttgcctgcatgacatcaccactattt

SEQ ID NO: 15377 - RNA, 2954 nt, Homo sapiens
  source 1..2954: mol_type = other RNA
gctgggattacaggcatgagccactgcgcctggcatgacaagtgattttcatactaaagttaattaaaatagacccaagaatcatatacaaacagggggaagagaggataaaaatgaccaagagcaactgaagccattcttgttgcaacttcctttccaaaggaaagcagaggcactgggagtgcagagatggcctcccgactccttgtcccagtgagaggcctgttgcgagccctgaccctttctcatcccaaaggcaaagctgaatctgggatgaggacaaggtacgtcctctggacctaggctatccccctaccctgtctctggctccaagtgggaagccagtcctgccctggcccagtgcagctgccaaggggacaaaaacagacccccagacacctttcagcttcgggtgaatcactttaatgctgttaacggcaagtctgtaaaaggttcaggacaaagttcttttttctttcttttttaattataaaactaacagctgttagaatctttttttctttttttccttttttcttttcccagctacaaaatactctggggagatgcattataatttaaaatatataatattgcacaaacaaccaaaaggttaattaaactaaagaaataattacaaagagaaaaaccccatcccgtcaaaaaaaagattcagcattctctccatcccaccccctcactgaaggtttgaagtggaagtgacctcactctctcggtgtccctgacccacgatccctttcactcattggtgagcacaccagattaggtacaagaatcaccagagcagcatcgtgaagcaccaggctctccagagattcctgcagcccctcattcccccagaggtgcagctttaccagagtggagggtgagagcacaaaggctgggtctgtcttcaggaagaagagcttttgcagaagcctgatgagagtttcaagttcacccccaggatagcccttccagaagcagaagggctgaggcggagaagctaggcttaccagagttgtaagtactcggctttgatcaccgctctgtaccgctggtagctgttttgtgtcctaaactacaggggagttgaggtgggtagctggttggacaaggtatcctgccaggcaacacacagaagggcctgaagtagccccctcccttcttggggaggggaagaaacgcaagagcgaactcctgcaggtggcacagctgggctaaggacttgggtgcatccgacatgaagaagccctgggaaggcatggggacagaccagcgtgggctggaggaaaggaaggaggtgggtcagggtttggtctctggattctgaaccccaaaggagcctttccaggaatggaaaatgcctgggagggggagagtcccaagagaggcaaatttcccagagataagtgcctcttacccactgggataggaaccaaaatgtgttcactgtccctgtttagccaagggtaggtggcatggccctccctgcctgcttatgtatggacagagtatgttgtctcagcttcctccgagagagactggtggtttagcttctgtctacacaggcagaagggctagaactatcccttgggacttcccagcaggagtcctcaggaacagtgggtgttcagcagaaaaacacaggctcttctggtgaggaggataggtttcctctcccttgggtcatcctattgttggcacaagtcagagtttctggccgggatttagagagccccttcccaggtgtgagcagaggcccaagagggccagcagggagccaccagaatctgtgcccagagctctggttggcagaggagatttgggggaacattctcagtcttccagggctgggctgagacgagcgagggaggcgagagatgccatgggtgggggagctgctccctctggctccctcactcccagtcctcccactctacatcttccagctccccggaggcatccactttggaaagtgccatctgcacctcctcttcagtcatgtccaagtcaaagtctttctcccagtcctcactgatgtccgtgcttgagcctttctttccattgttggagggtgtagacttcccactatccgagttcagctcaaacacccgtaagtctgtgggcgcctcctccctcagagtctctactctggctggaggcctgggctctgggccgccggtgtggccagcaggcgttaggggcttggagtgaatagggggtgagggtccagtctcacccacatccacagccaggccctgttcctccaaggatgcctctagcagcttttgggacaggtccttgggtagcactcgtgcctcaggtgcagtggccgggttggcgatctgtgtcacgagggagatgctctcactgctctctgatggagtcacctctgctgggggctcaactgaagtcaccagattctcttcacaggggctctgggggccaggttctccttcagggaatgtagaaattttggccacaggaacctttgcctcttttggagatatgggtgaaatgcccatgagctcctcttcctcctcctcccagccgggctcttcagagatgctctgttccgcccgctgcttcagggcgtccctccgggcctgctcctgctctaactgatggactttatagaaataccgatgccagaattctgaatgggaaacagctgctggaaccatcttggtgtagagggcccggatggaggggctgcctacaaggagctctgagatctcccccttcttctcctccaagcagaactgggaaagccaggcgtcaaacaattccgggggcccatctggttcattacagtaggttgctgggtccgactgcaggctatagaggcgagccttctctttgactgcttggtagctctgctgcagccagctccgccaccatcccacgtcctccccttccgccatcttgcctgcatgacatcaccactattt

SEQ ID NO: 15378 - RNA, 3239 nt, Homo sapiens
  source 1..3239: mol_type = other RNA
gctgggattacaggcatgagccactgcgcctggcatgacaagtgattttcatactaaagttaattaaaatagacccaagaatcatatacaaacagggggaagagaggataaaaatgaccaagagcaactgaagccattcttgttgcaacttcctttccaaaggaaagcagaggcactgggagtgcagagatggcctcccgactccttgtcccagtgagaggcctgttgcgagccctgaccctttctcatcccaaaggcaaagctgaatctgggatgaggacaaggtacgtcctctggacctaggctatccccctaccctgtctctggctccaagtgggaagccagtcctgccctggcccagtgcagctgccaaggggacaaaaacagacccccagacacctttcagcttcgggtgaatcactttaatgctgttaacggcaagtctgtaaaaggttcaggacaaagttcttttttctttcttttttaattataaaactaacagctgttagaatctttttttctttttttccttttttcttttcccagctacaaaatactctggggagatgcattataatttaaaatatataatattgcacaaacaaccaaaaggttaattaaactaaagaaataattacaaagagaaaaaccccatcccgtcaaaaaaaagattcagcattctctccatcccaccccctcactgaaggtttgaagtggaagtgacctcactctctcggtgtccctgacccacgatccctttcactcattggtgagcacaccagattaggtacaagaatcaccagagcagcatcgtgaagcaccaggctctccagagattcctgcagcccctcattcccccagaggtgcagctttaccagagtggagggtgagagcacaaaggctgggtctgtcttcaggaagaagagcttttgcagaagcctgatgagagtttcaagttcacccccaggatagcccttccagaagcagaagggctgaggcggagaagctaggcttaccagagttgtaagtactcggctttgatcaccgctctgtaccgctggtagctgttttgtgtcctaaactacaggggagttgaggtgggtagctggttggacaaggtatcctgccaggcaacacacagaagggcctgaagtagccccctcccttcttggggaggggaagaaacgcaagagcgaactcctgcaggtggcacagctgggctaaggacttgggtgcatccgacatgaagaagccctgggaaggcatggggacagaccagcgtgggctggaggaaaggaaggaggtgggtcagggtttggtctctggattctgaaccccaaaggagcctttccaggaatggaaaatgcctgggagggggagagtcccaagagaggcaaatttcccagagataagtgcctcttacccactgggataggaaccaaaatgtgttcactgtccctgtttagccaagggtaggtggcatggccctccctgcctgcttatgtatggacagagtatgttgtctcagcttcctccgagagagactggtggtttagcttctgtctacacaggcagaagggctagaactatcccttgggacttcccagcaggagtcctcaggaacagtgggtgttcagcagaaaaacacaggctcttctggtgaggaggataggtttcctctcccttgggtcatcctattgttggcacaagtcagagtttctggccgggatttagagagccccttcccaggtgtgagcagaggcccaagagggccagcagggagccaccagaatctgtgcccagagctctggttggcagaggagatttgggggaacattctcagtcttccagggctgggctgagacgagcgagggaggcgagagatgccatgggtgggggagctgctccctctggctccctcactcccagtcctcccactctacatcttccagctccccggaggcatccactttggaaagtgccatctgcacctcctcttcagtcatgtccaagtcaaagtctttctcccagtcctcactgatgtccgtgcttgagcctttctttccattgttggagggtgtagacttcccactatccgagttcagctcaaacacccgtaagtctgtgggcgcctcctccctcagagtctctactctggctggaggcctgggctctgggccgccggtgtggccagcaggcgttaggggcttggagtgaatagggggtgagggtccagtctcacccacatccacagccaggccctgttcctccaaggatgcctctagcagcttttgggacaggtccttgggtagcactcgtgcctcaggtgcagtggccgggttggcgatctgtgtcacgagggagatgctctcactgctctctgatggagtcacctctgctgggggctcaactgaagtcaccagattctcttcacaggggctctgggggccaggttctccttcagggaatgtagaaattttggccacaggaacctttgcctcttttggagatatgggtgaaatgcccatgagctcctcttcctcctcctcccagccgggctcttcagagatgctctgttccgcccgctgcttcagggcgtccctccgggcctgctcctgctctaactgatggactttatagaaataccgatgccagaattctgaatgggaaacagctgctggaaccatcttggtgtagagggcccggatggaggggctgcctacaaggagctctgagatctcccccttcttctcctccaagcagaactgggaaagccaggcgtcaaacaattccgggggcccatctggttcattacagtaggttgctgggtccgactgcaggctatagaggcgagccttggtgccatcatagggctcagctgtgccagacggtgtgcccatcagggtgatgacatcgcagtcgatggttttgtctggcgaaggggcaaaggtgtctgagatcacccctaggaagtcagataaccctttcttcatcttctctgttgctcctgaggagccttccgtagccagcttctccttgaccacgctggccgtggctgcgatggtacaggccgtgtcatgctgcaccacctgggtaaactccgtcaggtcccgcttcataaactccaaggcttcagaggacttctctttgactgcttggtagctctgctgcagccagctccgccaccatcccacgtcctccccttccgccatcttgcctgcatgacatcaccactattt

SEQ ID NO: 15379 - RNA, 3290 nt, Homo sapiens
  source 1..3290: mol_type = other RNA
gctgggattacaggcatgagccactgcgcctggcatgacaagtgattttcatactaaagttaattaaaatagacccaagaatcatatacaaacagggggaagagaggataaaaatgaccaagagcaactgaagccattcttgttgcaacttcctttccaaaggaaagcagaggcactgggagtgcagagatggcctcccgactccttgtcccagtgagaggcctgttgcgagccctgaccctttctcatcccaaaggcaaagctgaatctgggatgaggacaaggtacgtcctctggacctaggctatccccctaccctgtctctggctccaagtgggaagccagtcctgccctggcccagtgcagctgccaaggggacaaaaacagacccccagacacctttcagcttcgggtgaatcactttaatgctgttaacggcaagtctgtaaaaggttcaggacaaagttcttttttctttcttttttaattataaaactaacagctgttagaatctttttttctttttttccttttttcttttcccagctacaaaatactctggggagatgcattataatttaaaatatataatattgcacaaacaaccaaaaggttaattaaactaaagaaataattacaaagagaaaaaccccatcccgtcaaaaaaaagattcagcattctctccatcccaccccctcactgaaggtttgaagtggaagtgacctcactctctcggtgtccctgacccacgatccctttcactcattggtgagcacaccagattaggtacaagaatcaccagagcagcatcgtgaagcaccaggctctccagagattcctgcagcccctcattcccccagaggtgcagctttaccagagtggagggtgagagcacaaaggctgggtctgtcttcaggaagaagagcttttgcagaagcctgatgagagtttcaagttcacccccaggatagcccttccagaagcagaagggctgaggcggagaagctaggcttaccagagttgtaagtactcggctttgatcaccgctctgtaccgctggtagctgttttgtgtcctaaactacaggggagttgaggtgggtagctggttggacaaggtatcctgccaggcaacacacagaagggcctgaagtagccccctcccttcttggggaggggaagaaacgcaagagcgaactcctgcaggtggcacagctgggctaaggacttgggtgcatccgacatgaagaagccctgggaaggcatggggacagaccagcgtgggctggaggaaaggaaggaggtgggtcagggtttggtctctggattctgaaccccaaaggagcctttccaggaatggaaaatgcctgggagggggagagtcccaagagaggcaaatttcccagagataagtgcctcttacccactgggataggaaccaaaatgtgttcactgtccctgtttagccaagggtaggtggcatggccctccctgcctgcttatgtatggacagagtatgttgtctcagcttcctccgagagagactggtggtttagcttctgtctacacaggcagaagggctagaactatcccttgggacttcccagcaggagtcctcaggaacagtgggtgttcagcagaaaaacacaggctcttctggtgaggaggataggtttcctctcccttgggtcatcctattgttggcacaagtcagagtttctggccgggatttagagagccccttcccaggtgtgagcagaggcccaagagggccagcagggagccaccagaatctgtgcccagagctctggttggcagaggagatttgggggaacattctcagtcttccagggctgggctgagacgagcgagggaggcgagagatgccatgggtgggggagctgctccctctggctccctcactcccagtcctcccactctacatcttccagctccccggaggcatccactttggaaagtgccatctgcacctcctcttcagtcatgtccaagtcaaagtctttctcccagtcctcactgatgtccgtgcttgagcctttctttccattgttggagggtgtagacttcccactatccgagttcagctcaaacacccgtaagtctgtgggcgcctcctccctcagagtctctactctggctggaggcctgggctctgggccgccggtgtggccagcaggcgttaggggcttggagtgaatagggggtgagggtccagtctcacccacatccacagccaggccctgttcctccaaggatgcctctagcagcttttgggacaggtccttgggtagcactcgtgcctcaggtgcagtggccgggttggcgatctgtgtcacgagggagatgctctcactgctctctgatggagtcacctctgctgggggctcaactgaagtcaccagattctcttcacaggggctctgggggccaggttctccttcagggaatgtagaaattttggccacaggaacctttgcctcttttggagatatgggtgaaatgcccatgagctcctcttcctcctcctcccagccgggctcttcagagatgctctgttccgcccgctgcttcagggcgtccctccgggcctgctcctgctctaactgatggactttatagaaataccgatgccagaattctgaatgggaaacagctgctggaaccatcttggtgtagagggcccggatggaggggctgcctacaaggagctctgagatctcccccttcttctcctccaagcagaactgggaaagccaggcgtcaaacaattccgggggcccatctggttcattacagtaggttgctgggtccgactgcaggctatagaggcgagccttggtgccatcatagggctcagctgtgccagacggtgtgcccatcagggtgatgacatcgcagtcgatggttttgtctggcgaaggggcaaaggtgtctgagatcacccctaggaagtcagataaccctttcttcatcttctctgttgctcctgaggagccttccgtctgtatagagaacgggcagaggaagcaagcgccccgggaacaggctgcaatagccagcttctccttgaccacgctggccgtggctgcgatggtacaggccgtgtcatgctgcaccacctgggtaaactccgtcaggtcccgcttcataaactccaaggcttcagaggacttctctttgactgcttggtagctctgctgcagccagctccgccaccatcccacgtcctccccttccgccatcttgcctgcatgacatcaccactattt

SEQ ID NO: 15380 - RNA, 5082 nt, Homo sapiens
  source 1..5082: mol_type = other RNA
gctgggattacaggcatgagccactgcgcctggcatgacaagtgattttcatactaaagttaattaaaatagacccaagaatcatatacaaacagggggaagagaggataaaaatgaccaagagcaactgaagccattcttgttgcaacttcctttccaaaggaaagcagaggcactgggagtgcagagatggcctcccgactccttgtcccagtgagaggcctgttgcgagccctgaccctttctcatcccaaaggcaaagctgaatctgggatgaggacaaggtacgtcctctggacctaggctatccccctaccctgtctctggctccaagtgggaagccagtcctgccctggcccagtgcagctgccaaggggacaaaaacagacccccagacacctttcagcttcgggtgaatcactttaatgctgttaacggcaagtctgtaaaaggttcaggacaaagttcttttttctttcttttttaattataaaactaacagctgttagaatctttttttctttttttccttttttcttttcccagctacaaaatactctggggagatgcattataatttaaaatatataatattgcacaaacaaccaaaaggttaattaaactaaagaaataattacaaagagaaaaaccccatcccgtcaaaaaaaagattcagcattctctccatcccaccccctcactgaaggtttgaagtggaagtgacctcactctctcggtgtccctgacccacgatccctttcactcattggtgagcacaccagattaggtacaagaatcaccagagcagcatcgtgaagcaccaggctctccagagattcctgcagcccctcattcccccagaggtgcagctttaccagagtggagggtgagagcacaaaggctgggtctgtcttcaggaagaagagcttttgcagaagcctgatgagagtttcaagttcacccccaggatagcccttccagaagcagaagggctgaggcggagaagctaggcttaccagagttgtaagtactcggctttgatcaccgctctgtaccgctggtagctgttttgtgtcctaaactacaggggagttgaggtgggtagctggttggacaaggtatcctgccaggcaacacacagaagggcctgaagtagccccctcccttcttggggaggggaagaaacgcaagagcgaactcctgcaggtggcacagctgggctaaggacttgggtgcatccgacatgaagaagccctgggaaggcatggggacagaccagcgtgggctggaggaaaggaaggaggtgggtcagggtttggtctctggattctgaaccccaaaggagcctttccaggaatggaaaatgcctgggagggggagagtcccaagagaggcaaatttcccagagataagtgcctcttacccactgggataggaaccaaaatgtgttcactgtccctgtttagccaagggtaggtggcatggccctccctgcctgcttatgtatggacagagtatgttgtctcagcttcctccgagagagactggtggtttagcttctgtctacacaggcagaagggctagaactatcccttgggacttcccagcaggagtcctcaggaacagtgggtgttcagcagaaaaacacaggctcttctggtgaggaggataggtttcctctcccttgggtcatcctattgttggcacaagtcagagtttctggccgggatttagagagccccttcccaggtgtgagcagaggcccaagagggccagcagggagccaccagaatctgtgcccagagctctggttggcagaggagatttgggggaacattctcagtcttccagggctgggctgagacgagcgagggaggcgagagatgccatgggtgggggagctgctccctctggctccctcactcccagtcctcccactctacatcttccagctgcaaatgggagggggtaatggaaatcacaaacacatagttactcctgagtcaggcccagacctaacctccacttgctgagcagagccacctcccatcccctaccccaggccatactctgaggtcccactgagagtgaacccctagtcttaaggaatgtgtctgaggggcagagctgccctctgcctgaggggtgggcctgatgctctgattacctcagacctaaaggaaacacttcccccaaccaacaccagacaccacaaggtgatggctgcctacaggaaccaagtcagcctcagtcctttaaggagaacttgcctcctgctgagcagataatgccatggctctgagaagcagagaactcaggaggcctgagcagatacttggccctggacacaaaagaccagtgtaatcaagggcaagttacttagtctttgggtgaatggaggccactgcctgagtggcactgtggccaaaagcagaggtggcagtggcctacagatgcccactaggtcttcactaggggcaccaacaccctaattcccagctcaagtctccccacggaacgttttcttgctttgttcctactcttggcctgctgtcggctaagccctggtatagcaggttctagaatgctcacgtgtactgcacgtcaggttttaaagggggctgcaaagacacaaaaagccagcaagcccctgtggcctgacagggcactatgggctttctctgtcctgggtatagtgaggtagtcacaagtgcaaaatactcctgagtaggtaaaatactcccccaaggcttcagtttcccatcatgaaaaaggaggcccttcacatgtctctctaatctgtccacctctttctaacaggctcataagttacatgatggaaggactcatgtggttcttatgtgacagtggaactaacgctgacatgaatcagatgtctgggttgcagcctcagtcctgtcacttattagctgggagagctttggactgttccagcctctcaatctaaatgagccacttttgattctgagaggtagtgaagaataacagtactaaggcctccttgagcttaataactggaatgggttttgtggggtttatcactaatgtctcctgagtgctggtcaccatgtctcaggcaatagccctaaggtgtctacatggatcacctcattacagcttatagccaggtcttataatgatcaattccatgttttagatgaggaaccaggggctcaggttaagtaacttgcccttgcccttgatcacactggtcttttgtctccaaggccaagtatatactcaggcctcatacctgaggaccacaactcagaaggtcaggcagggtttgatgtctgttttcttttttcctttttttttttttttcaaaaacagaaatggggtctcactatattggccaggctggtcttgaactcctcgcctcaagcaatcctcccaccttggcctcccaaagtgttgggattacaggtgtgagccaccgcgctcagcatgacatctgttttcttaagcagtttctcaggcaattttgatacagagctaaggtcaagaacttgaccctctatccaccctggaactgaggaaaagtgcagcctgctgatgaccaatgttgtgggtctgagcaggaagctccagctcctttcccaccacctgtcacctcagacaggagcagggaccctcctgaggggacagctgggctggctggggagagctctcacacccaggaccattaggctcgcttccctctgacccaccaggcccactcacctccccggaggcatccactttggaaagtgccatctgcacctcctcttcagtcatgtccaagtcaaagtctttctcccagtcctcactgatgtccgtgcttgagcctttctttccattgttggagggtgtagacttcccactatccgagttcagctcaaacacccgtaagtctgtgggcgcctcctccctcagagtctctactctggctggaggcctgggctctgggccgccggtgtggccagcaggcgttaggggcttggagtgaatagggggtgagggtccagtctcacccacatccacagccaggccctgttcctccaaggatgcctctagcagcttttgggacaggtccttgggtagcactcgtgcctcaggtgcagtggccgggttggcgatctgtgtcacgagggagatgctctcactgctctctgatggagtcacctctgctgggggctcaactgaagtcaccagattctcttcacaggggctctgggggccaggttctccttcagggaatgtagaaattttggccacaggaacctttgcctcttttggagatatgggtgaaatgcccatgagctcctcttcctcctcctcccagccgggctcttcagagatgctctgttccgcccgctgcttcagggcgtccctccgggcctgctcctgctctaactgatggactttatagaaataccgatgccagaattctgaatgggaaacagctgctggaaccatcttggtgtagagggcccggatggaggggctgcctacaaggagctctgagatctcccccttcttctcctccaagcagaactgggaaagccaggcgtcaaacaattccgggggcccatctggttcattacagtaggttgctgggtccgactgcaggctatagaggcgagccttggtgccatcatagggctcagctgtgccagacggtgtgcccatcagggtgatgacatcgcagtcgatggttttgtctggcgaaggggcaaaggtgtctgagatcacccctaggaagtcagataaccctttcttcatcttctctgttgctcctgaggagccttccgtctgtatagagaacgggcagaggaagcaagcgccccgggaacaggctgcaatagccagcttctccttgaccacgctggccgtggctgcgatggtacaggccgtgtcatgctgcaccacctgggtaaactccgtcaggtcccgcttcataaactccaaggcttcagaggacttctctttgactgcttggtagctctgctgcagccagctccgccaccatcccacgtcctccccttccgccatcttgcctgcatgacatcaccactattt

SEQ ID NO: 15381 - RNA, 1457 nt, Homo sapiens
  source 1..1457: mol_type = other RNA
gctgggattacaggcatgagccactgcgcctggccaagacatggcatcttaagtccaattttcagggcaggaggcaaaagtggcatcaccctggtgggcgagtgggggtggggggaaaacacttttgttgttggctaaaaagcctgcattttaaccaaagggaatataaattactctgtgcccaaactagcactatttaaaaaaaaaaaaaaagagagagagagaagaaagaaagcaagaaagaaagaaagcaagaaagaaagaaagaaagaaagaaagaaagccagccagccagccatatcccagggtggccccagaaagggccaggctgttgagcacagttcaaggtcgaggacgcattgagaggcttttaaatttggtaaaagccagtcttggatataaaatgaattctgaaattccttcaccaacggacaggaaagcaggtgaacatatggccccagccgtggtatcgcagctcatggattcaccagaccaagattctccctgggcatctggacctcccaggctggcctccctggtcacggcagctgtgtccccagatgcagggaggaaaatgggagaaaaaaaaattttcaccacttccctcgaatcaaccggagcttttgtagagaaggaggaagaggaggtgggcagatcagaatctctcttccagatcggatccccaagctgaagagcttgtcttttcctggccacaccccagagggtggatgtcccctcgtggggtccccagcaggatgaggtcttaggagacctgagcgtccctcagtgtttgtggcaatagttgattttgccctctgactgctccaggaggtccaacatctcctcaatgatggctctcagtgccctgcccagctggtccgcgttgtacggcttccccagtgggggcacgtggacgaaggctgatcgaccgtgactctgccggcatcctgcgagatggtcaccgacacatccaggcccaacgtggtgactcgcttgcacacagcatccatgtcgatgatggagtcaatgctttcaggcccgtcctccacgcagcactgggagccggggcaaaagcggcagttgtccagccccttgtagcccttgttgtgtccacatttctccagtgtgactgtggtcgccatgcctgacacccccacatgcaccaccagctgtggactgtgcttctcccacagggcggggatgagtctctggactgtttggtactcaaccggaatctcgtacacatgcaggtccacgctgtcgccaaggcctagcttttctagctcctgaactgcaatccaactggcgttcacggtgtgttccccaaaagggccaaatcccgtcactaccaccgccttcctcggctgctccatggcgggatcgggctgtgcctcggacctgcttctgttgcgactggcgcgacagctgctgccgctgcagcctctcggccgcgcgag

SEQ ID NO: 15382 - RNA, 1578 nt, Homo sapiens
  source 1..1578: mol_type = other RNA
gctgggattacaggcatgagccactgcgcctggccaagacatggcatcttaagtccaattttcagggcaggaggcaaaagtggcatcaccctggtgggcgagtgggggtggggggaaaacacttttgttgttggctaaaaagcctgcattttaaccaaagggaatataaattactctgtgcccaaactagcactatttaaaaaaaaaaaaaaagagagagagagaagaaagaaagcaagaaagaaagaaagcaagaaagaaagaaagaaagaaagaaagaaagccagccagccagccatatcccagggtggccccagaaagggccaggctgttgagcacagttcaaggtcgaggacgcattgagaggcttttaaatttggtaaaagccagtcttggatataaaatgaattctgaaattccttcaccaacggacaggaaagcaggtgaacatatggccccagccgtggtatcgcagctcatggattcaccagaccaagattctccctgggcatctggacctcccaggctggcctccctggtcacggcagctgtgtccccagatgcagggaggaaaatgggagaaaaaaaaattttcaccacttccctcgaatcaaccggagcttttgtagagaaggaggaagaggaggtgggcagatcagaatctctcttccagatcggatccccaagctgaagagcttgtcttttcctggccacaccccagagggtggatgtcccctcgtggggtccccagcaggatgaggtcttaggagacctgagcgtccctcagtgtttgtggcaatagttgattttgccctctgactgctccaggaggtccaacatctcctcaatgatggctctcagtgccctgcccagctggtccgcgttgtacggcttccccagtgggggcacgtggacgaaggctgatcgaccgtgactctgccggcatcctgcgagatggtcaccgacacatccaggcccaacgtggtgactcgcttgcacacagcatccatgtcgatgatggagtcaatgctttcaggcccgtcctccacgcagcactgggagccggggcaaaagcggcagttgtccagccccttgtagcccttgttgtgtccacatttctccagtgtgactgtggtcgccatgcctgacacccccacatgcaccaccagctgtggactgtgcttctcccacagggcggggatgagtctctggactgtttggtactcaaccggaatctcgtacacatgcaggtccacgctgtcgccaaggcctagcttttctagctcctgatggcagggctcggtggctcacacctataatcccagcttctttgggaggccgaggtggaaggatcatttgagcccggaagttcaagaccagccagggcaatatagtgagatcccatctctgaactgcaatccaactggcgttcacggtgtgttccccaaaagggccaaatcccgtcactaccaccgccttcctcggctgctccatggcgggatcgggctgtgcctcggacctgcttctgttgcgactggcgcgacagctgctgccgctgcagcctctcggccgcgcgag

SEQ ID NO: 15383 - RNA, 1444 nt, Homo sapiens
  source 1..1444: mol_type = other RNA
gctgggattacaggcatgagccactgcgcctggccaagacatggcatcttaagtccaattttcagggcaggaggcaaaagtggcatcaccctggtgggcgagtgggggtggggggaaaacacttttgttgttggctaaaaagcctgcattttaaccaaagggaatataaattactctgtgcccaaactagcactatttaaaaaaaaaaaaaaagagagagagagaagaaagaaagcaagaaagaaagaaagcaagaaagaaagaaagaaagaaagaaagaaagccagccagccagccatatcccagggtggccccagaaagggccaggctgttgagcacagttcaaggtcgaggacgcattgagaggcttttaaatttggtaaaagccagtcttggatataaaatgaattctgaaattccttcaccaacggacaggaaagcaggtgaacatatggccccagccgtggtatcgcagctcatggattcaccagaccaagattctccctgggcatctggacctcccaggctggcctccctggtcacggcagctgtgtccccagatgcagggaggaaaatgggagaaaaaaaaattttcaccacttccctcgaatcaaccggagcttttgtagagaaggaggaagaggaggtgggcagatcagaatctctcttccagatcggatccccaagctgaagagcttgtcttttcctggccacaccccagagggtggatgtcccctcgtggggtccccagcaggatgaggtcttaggagacctgagcgtccctcagtgtttgtggcaatagttgattttgccctctgactgctccaggaggtccaacatctcctcaatgatggctctcagtgccctgcccagctggtccgcgttgtacggcttccccagtgggggcacgtggacgaaggctgatcgaccgtgactctggtacaaagaggtgtagtaggtaaagtcgcagagatatctgccggcatcctgcgagatggtcaccgacacatccaggcccaacgtggtgactcgcttgcacacagcatccatgtcgatgatggagtcaatgctttcaggcccgtcctccacgcagcactgggagccggggcaaaagcggcagttgtccagccccttgtagcccttgttgtgtccacatttctccagtgtgactgtggtcgccatgcctgacacccccacatgcaccaccagctgtggactgtgcttctcccacagggcggggatgagtctctggactgtttggtactcaaccggaatctcgtacacatgcaggtccacgctgtcgccaaggcctagcttttctagctcccgtcactaccaccgccttcctcggctgctccatggcgggatcgggctgtgcctcggacctgcttctgttgcgactggcgcgacagctgctgccgctgcagcctctcggccgcgcgag

SEQ ID NO: 15384 - RNA, 1497 nt, Homo sapiens
  source 1..1497: mol_type = other RNA
gctgggattacaggcatgagccactgcgcctggccaagacatggcatcttaagtccaattttcagggcaggaggcaaaagtggcatcaccctggtgggcgagtgggggtggggggaaaacacttttgttgttggctaaaaagcctgcattttaaccaaagggaatataaattactctgtgcccaaactagcactatttaaaaaaaaaaaaaaagagagagagagaagaaagaaagcaagaaagaaagaaagcaagaaagaaagaaagaaagaaagaaagaaagccagccagccagccatatcccagggtggccccagaaagggccaggctgttgagcacagttcaaggtcgaggacgcattgagaggcttttaaatttggtaaaagccagtcttggatataaaatgaattctgaaattccttcaccaacggacaggaaagcaggtgaacatatggccccagccgtggtatcgcagctcatggattcaccagaccaagattctccctgggcatctggacctcccaggctggcctccctggtcacggcagctgtgtccccagatgcagggaggaaaatgggagaaaaaaaaattttcaccacttccctcgaatcaaccggagcttttgtagagaaggaggaagaggaggtgggcagatcagaatctctcttccagatcggatccccaagctgaagagcttgtcttttcctggccacaccccagagggtggatgtcccctcgtggggtccccagcaggatgaggtcttaggagacctgagcgtccctcagtgtttgtggcaatagttgattttgccctctgactgctccaggaggtccaacatctcctcaatgatggctctcagtgccctgcccagctggtccgcgttgtacggcttccccagtgggggcacgtggacgaaggctgatcgaccgtgactctggtacaaagaggtgtagtaggtaaagtcgcagagatatctgccggcatcctgcgagatggtcaccgacacatccaggcccaacgtggtgactcgcttgcacacagcatccatgtcgatgatggagtcaatgctttcaggcccgtcctccacgcagcactgggagccggggcaaaagcggcagttgtccagccccttgtagcccttgttgtgtccacatttctccagtgtgactgtggtcgccatgcctgacacccccacatgcaccaccagctgtggactgtgcttctcccacagggcggggatgagtctctggactgtttggtactcaaccggaatctcgtacacatgcaggtccacgctgtcgccaaggcctagcttttctagctcctgaactgcaatccaactggcgttcacggtgtgttccccaaaagggccaaatcccgtcactaccaccgccttcctcggctgctccatggcgggatcgggctgtgcctcggacctgcttctgttgcgactggcgcgacagctgctgccgctgcagcctctcggccgcgcgag

SEQ ID NO: 15385 - RNA, 1618 nt, Homo sapiens
  source 1..1618: mol_type = other RNA
gctgggattacaggcatgagccactgcgcctggccaagacatggcatcttaagtccaattttcagggcaggaggcaaaagtggcatcaccctggtgggcgagtgggggtggggggaaaacacttttgttgttggctaaaaagcctgcattttaaccaaagggaatataaattactctgtgcccaaactagcactatttaaaaaaaaaaaaaaagagagagagagaagaaagaaagcaagaaagaaagaaagcaagaaagaaagaaagaaagaaagaaagaaagccagccagccagccatatcccagggtggccccagaaagggccaggctgttgagcacagttcaaggtcgaggacgcattgagaggcttttaaatttggtaaaagccagtcttggatataaaatgaattctgaaattccttcaccaacggacaggaaagcaggtgaacatatggccccagccgtggtatcgcagctcatggattcaccagaccaagattctccctgggcatctggacctcccaggctggcctccctggtcacggcagctgtgtccccagatgcagggaggaaaatgggagaaaaaaaaattttcaccacttccctcgaatcaaccggagcttttgtagagaaggaggaagaggaggtgggcagatcagaatctctcttccagatcggatccccaagctgaagagcttgtcttttcctggccacaccccagagggtggatgtcccctcgtggggtccccagcaggatgaggtcttaggagacctgagcgtccctcagtgtttgtggcaatagttgattttgccctctgactgctccaggaggtccaacatctcctcaatgatggctctcagtgccctgcccagctggtccgcgttgtacggcttccccagtgggggcacgtggacgaaggctgatcgaccgtgactctggtacaaagaggtgtagtaggtaaagtcgcagagatatctgccggcatcctgcgagatggtcaccgacacatccaggcccaacgtggtgactcgcttgcacacagcatccatgtcgatgatggagtcaatgctttcaggcccgtcctccacgcagcactgggagccggggcaaaagcggcagttgtccagccccttgtagcccttgttgtgtccacatttctccagtgtgactgtggtcgccatgcctgacacccccacatgcaccaccagctgtggactgtgcttctcccacagggcggggatgagtctctggactgtttggtactcaaccggaatctcgtacacatgcaggtccacgctgtcgccaaggcctagcttttctagctcctgatggcagggctcggtggctcacacctataatcccagcttctttgggaggccgaggtggaaggatcatttgagcccggaagttcaagaccagccagggcaatatagtgagatcccatctctgaactgcaatccaactggcgttcacggtgtgttccccaaaagggccaaatcccgtcactaccaccgccttcctcggctgctccatggcgggatcgggctgtgcctcggacctgcttctgttgcgactggcgcgacagctgctgccgctgcagcctctcggccgcgcgag

SEQ ID NO: 15386 - RNA, 1264 nt, Homo sapiens
  source 1..1264: mol_type = other RNA
gctgggattacaggcatgagccactgcgcctggccaagacatggcatcttaagtccaattttcagggcaggaggcaaaagtggcatcaccctggtgggcgagtgggggtggggggaaaacacttttgttgttggctaaaaagcctgcattttaaccaaagggaatataaattactctgtgcccaaactagcactatttaaaaaaaaaaaaaaagagagagagagaagaaagaaagcaagaaagaaagaaagcaagaaagaaagaaagaaagaaagaaagaaagccagccagccagccatatcccagggtggccccagaaagggccaggctgttgagcacagttcaaggtcgaggacgcattgagaggcttttaaatttggtaaaagccagtcttggatataaaatgaattctgaaattccttcaccaacggacaggaaagcaggtgaacatatggccccagccgtggtatcgcagctcatggattcaccagaccaagattctccctgggcatctggacctcccaggctggcctccctggtcacggcagctgtgtccccagatgcagggaggaaaatgggagaaaaaaaaattttcaccacttccctcgaatcaaccggagcttttgtagagaaggaggaagaggaggtgggcagatcagaatctctcttccagatcggatccccaagctgaagagcttgtcttttcctggccacaccccagagggtggatgtcccctcgtggggtccccagcaggatgaggtcttaggagacctgagcgtccctcagtgtttgtggcaatagttgattttgccctctgactgctccaggaggtccaacatctcctcaatgatggctctcagtgccctgcccagctggtccgcgttgtacggcttccccagtgggggcacgtggacgaaggctgatcgaccgtgactctggtacaaagaggtgtagtaggtaaagtcgcagagatatctgtggactgtgcttctcccacagggcggggatgagtctctggactgtttggtactcaaccggaatctcgtacacatgcaggtccacgctgtcgccaaggcctagcttttctagctcctgaactgcaatccaactggcgttcacggtgtgttccccaaaagggccaaatcccgtcactaccaccgccttcctcggctgctccatggcgggatcgggctgtgcctcggacctgcttctgttgcgactggcgcgacagctgctgccgctgcagcctctcggccgcgcgag

SEQ ID NO: 15387 - RNA, 1637 nt, Homo sapiens
  source 1..1637: mol_type = other RNA
gctgggattacaggcatgagccactgcgcctggccaatgaacaagtgtttcagtgccactgacaaaccaagactcccctaatcttgaagccactgccttcccctgacagatgagaaatctgagacccagagagggcaaatcacatgtccaaccccacacagactgtctgtggtagagccagggctggtaccctggtttcccactgctggccggaactccttctgcaaacccaggctaccttgccacagtgctttccttgcagtttctgcaaaatggccgagtgagactcccccacagcctcctcccgctgtcatccctccagcgagacaaaaggcaatttaccgaaatgttataatcacctggaggctggcacgcggggacatccatgctttatctgcggtgttgttagcagcaccgtaatgaaggctttgtggagggataatacgctgtaactgccaaatcaaatgcccgcaccaatcacacatccctgccagcagacgcgcatttgtctcaatgtagccgtgcagggtgaccatgcgcgcccgctcggggctgctgaacggggtgtagtggatgtcgtcggacagggcggagggaaggcgggacgggggcgcccccgagggcggcactgggtgttgcggcgtgtgctttttatgacgcgcccggcagttttgaaaccacacctggatgactctccggctgaggcccgtcatgtccgccagcttctgcagcgtctgagcgtcggggttgttgtcctgcgcgaactgcgcctgcataacctgcagctgttccgcggtgaaggacgtccgcgcgcgcttggccggcttgggttgactgtcctgttccgagggcactgccccctccaacgtgaggccgttcccgttctcggcggccctcttgaggttctcaatcatggtgtcgtagtggatgcggcagagcaccttctcctcgaccaggccgaactcctcaccagtggacagctggcgcttgcacgagaagcaggcgaagcaggccaggtggtaggcgttgccgcgagctctccgcacccagtcgctggcgtagatctgtcggccgcaccgggcacacttggtcccgaatcggctgaagtagtccatcttgcagaagatctccttgttcttgatgtagcagctgttctgctgcctcagcgacgtgcgacacacggagcactcgaggcaccgcacgtgccagatgaggttgttgaccttgagcagatatcggtccaggatctcgaggccgcagctggagcagatgttcttgcctgcagacggcacggaggaggcggcagagggcggtgagcagacagatggcgtgctgggcgtacatggggaggcctgaccctcgtccttgtccagagctcctgccagggcctcggcgtcagactgagccatggcgggcggcgcggtcccttcaagacagcgggtggtcgctttgcagccggaccctggctgggccatcacctgcaattagaaattgtcgtgaatgcccaagataagaggtagccagagtgtcaattccaactgtcaatcagtgagatccatcaggccgcccaaagaattgcaaatttgattttttaatggtagtaattaaaaatcgaattttttctctctccacccgcc

SEQ ID NO: 15388 - RNA, 1715 nt, Homo sapiens
  source 1..1715: mol_type = other RNA
gctgggattacaggcatgagccactgcgcctggccaatgaacaagtgtttcagtgccactgacaaaccaagactcccctaatcttgaagccactgccttcccctgacagatgagaaatctgagacccagagagggcaaatcacatgtccaaccccacacagactgtctgtggtagagccagggctggtaccctggtttcccactgctggccggaactccttctgcaaacccaggctaccttgccacagtgctttccttgcagtttctgcaaaatggccgagtgagactcccccacagcctcctcccgctgtcatccctccagcgagacaaaaggcaatttaccgaaatgttataatcacctggaggctggcacgcggggacatccatgctttatctgcggtgttgttagcagcaccgtaatgaaggctttgtggagggataatacgctgtaactgccaaatcaaatgcccgcaccaatcacacatccctgccagcagacgcgcatttgtctcaatgtagccgtgcagggtgaccatgcgcgcccgctcggggctgctgaacggggtgtagtggatgtcgtcggacagggcggagggaaggcgggacgggggcgcccccgagggcggcactgggtgttgcggcgtgtgctttttatgacgcgcccggcagttttgaaaccacacctggatgactctccggctgaggcccgtcatgtccgccagcttctgcagcgtctgagcgtcggggttgttgtcctgcgcgaactgcgcctgcataacctgcagctgttccgcggtgaaggacgtccgcgcgcgcttggccggcttgggttgactgtcctgttccgagggcactgccccctccaacgtgaggccgttcccgttctcggcggccctcttgaggttctcaatcatggtgtcgtagtggatgcggcagagcaccttctcctcgaccaggccgaactcctcaccagtggacagctggcgcttgcacgagaagcaggcgaagcaggccaggtggtaggcgttgccgcgagctctccgcacccagtcgctggcgtagatctgtcggccgcaccgggcacacttggtcccgaatcggctgaagtagtccatcttgcagaagatctccttgttcttgatgtagcagctgttctgctgcctcagcgacgtgcgacacacggagcactcgaggcaccgcacgtgccagatgaggttgttgaccttgagcagatatcggtccaggatctcgaggccgcagctggagcagatgttcttgcctgcagacggcacggaggaggcggcagagggcggtgagcagacagatggcgtgctgggcgtacatggggaggcctgaccctcgtccttgtccagagctcctgccagggcctcggcgtcagactgagccatggcgggcggcgcggtcccttcaagacagcgggtggtcgctttgcagccggaccctggctgggccatcacctggtcggtggcggggccgccctcggccggcagccggcagccctcgggcaacgccggggcggcgttctcatgcttccagtacatgggccggggaacctcgggctcagcgggcgcgcagcgcggagagctgcgccgagggggaccacagccgcagtgggagcagaggctgctgcaggagcaggaggagagccgaggcgccggccccgccgccccgggcccggcctcagcccccgcccc

SEQ ID NO: 15389 - RNA, 4783 nt, Homo sapiens
  source 1..4783: mol_type = other RNA
gctgggattacaggcatgagccactgcgcctggccaccaacagattttttaattcagaatttgacagcaaataagtgttacatcttttaaaacaaatagcttcaaagaaatatattaatgggaaaatattaaacatatcatttttattaaagtatatcaacacctagaaacaataaagggtacatgatgaatatgtataaaaacaagtaactcaaagctttacttgaaatagaaaagtctaactataagttattttttgtgtgcatcaattgaaacaaaccataagtttgttgattataatgtcattttatgcattgcaagaatatacaacttcaaagtcttctggtttaaattcctaaataactacagggtaactaaatatgttcaggatccttcaggcagaaaaatcaactatttagagtcacctggaacaaataaataagtaatcatgccacatttctgttgtttttaaatttatcatggttttgcttataaaggtattgactcattaggttaactctgtaagattataagatgatattctgatttatacttgctacatttatgactacttggagaaacaacacttgaaggggaccttctatatacatttgaacaatctgagttacaaataatcatgctgacaaattcaggtttccccactaccactgaaattatcagagtctaagctgaaaaaaaaaaatccaagtattgtattcatacattttaatcaaggttcaatagggaagaagggaagaaaaagtaaaattgcaaacaaaatgttaaatactgtactccacttcctctgaaatatttgtcttttgaattagtatactggtctaaattttgcctccaaaaatctaagaagaatattgtttgggtttttcaaaaatctacatacttcttgagtgttctattcaaattttatgtaatcagaaacctattttaaggcataaaattagaaaaaaatttaaaaattattaacttcaattaacctcaaataaatagaattgtattgtatgctccactgcctttgttctactcagctttttcagtttgcggtttaaagcctccatatttcttttcaatgtttaaaaagacatgctgttttcattttccctttcctttaaaaaatggcagaataatctattgaaaaacaaagaggcaaaaactccttgaactatttttcctctcctttaaaacagacctatatttggtgtatgtatcttttaagtttgcagtatgtgagaaagaggaccgtaatcataaagttctttttttaaaataactaggaatgacagagtgatttatccccatgggaagtgcaataaacatattgtatagtatatatgaccttatgctttacttggtgcccctaaaagactgaattatattcattgatctattttaatacagcaaactacaatttaacgttaaaacaaatttgatgctcaaagcacttctgtagaagatacaaaagataaatgtttgaatcttacccagatcactataggcaacaactaagcatataaactacagacataaataatacacaatccaggccaggtgtagtggctaacaccgtaatcccagcactttgggagaccaaggcgtgtggatcacttgcggtcaggagttcgagaccagcctgaccaacatggttgaaccctgtctctaccaaaaaaaaatacaaaatttgctgggcatggtggcacatgcctataatcccagctacttgggaggctgatacaggagaatcgcttgaagctgggaggcagaggttgcagtgagccaagatcacgccactgcactccagcctgggcaataagagcaaaactctgtctcaaataataataatatcattaagagcaaaactccatctcaaaaataataataatacatgagccattatgaacaaattctatcaaggcttcatgtgacatttaatggctgaaaactaaacaggatttagcaaaataaaatgtatttaaatacatcctttcttatgaaaggagaaggcttatccagtgatactgaccatagagagaacctatacatcagtctcatatttaagagggttctgcctgccttggttggcttcaaagagctcactgtacgttgattatatttagactgcttcttagcagaagcaaagagtttataacagttcataacatcacaagtgatggcatcttgtcacggtgtaagcaatctcaaaacataacttgcatttatcacttctactttttgctcatgacagcatatgaaagcctgccttctcaaatgcacagatgtgttcaatatgcactttccatctatgcttgctctttataatgtatatttaagaagagctcaagacttttaaaaataaaacctacatggcaatgatatcttctaagtcatgaaaaactatgtggaaactatcaggccaggcgtggtggctgatgcctgtaatcctagcacttgggaggctaaggcgggaggatcacttaagcctaggagtttgagatcagcctgggcaacatggcaagactcctgtctctacaaaaataaaaataaaattagccagatgtggtggcgcacagctgtagtctcagctactcaggagactgaggtgggaggactgcttgagcccaggaggtagaggctgcagtgcgttgtgttcatgccactccactctagcctaggtgacagagcaagaccctgtctcgaaaaaaaaaaaaaagaaaagaaaaaagaaactgtcttaattaattaattttaagtataccatattctgaagaaaaaatcaaaatctttaagcaaatttataatgtacagagctcagttcttcaaatacggagacattaaagaaaaaagaacctattcaaaggccaaagataaaactgtaaatgattgtgggtctcctaaaagtatatttaaagtttcttacaaaaccataacccttctcccctaaaaaatatgttctctggtagaatactgaagtagaaaacagaccactaaacaatgatcttgcagtatcaaacattttctcaaaaaattatgacataggatcaaaaaaacagaatgctaggcacccaagataaaaagcacaaaatgtaagagaatagatcacctgttcaaagaaccaaagctcacaataacgtatgacagaacacctatacattaaaaaaaaaaagaaagaaatgccgataacagaattgaaaaaaacaaaatgaggtcggatgcagtggctcacgcctgtaatcccagtatttagagaggccaaggtgggtggatcacctgaggtcaggagttcgagactgcctggcctatgtggtgagactccatctctactaaaaacacaaaaattagctgggcatggtggcaggcacctataatcccagctatatgggaggctggggcaggagaatcgcttgaacccgggaggcagaggttgcagtgagctgagattgcgccattgcactccagcctgggtgacaagagccaaactccatctaaaaaaagaaaaaaaaagaagaagacaaaatgaaaagtgtatatttttcataagagaacataagaattttgtgaatattgtagccactgtgtaaatattgtataaaccttcagatactggttatctcttttgggagatttaaggtattcatttttaatcttaaaaagattctttaaaaagaaatatacttccctttgaaatagtaagttaagtagcatttcaagtttttctttcataaaaacagttgctggaacagaaaaataggcttcattaaatgattctctccatgctctaaatacacattttaaatttaaacctttttcttctacagaaagcaatgattactaacactttgttattttcccttagcaatttaaaaaagcatttaatcacacattataataacaaagagaaagtaatgacatttgaaatttacttatacagtaggtcaggacaatcaaattgacctccatttatgcataaaaaaggcaagagaaaaaagggagttttgctagtctactctccaaaaaagggaaaagatggctatagaagtcaattcagaaactacagttgtccattgtctgctacaatgcaactcatgaactgttctcctgtattctgtcacacttattgctttctttgccctcttgatatgtacgaagctgctccatgaagccagaatttggacatatggaaggtcttgcatttttcaccaaagaaaaagcactggtaaatgaggtttgttcagaattcatcaggaaacctattacaattgcagcagccctggaaacgcctgcattacaatgaacaagaaccactccatccttattctttttcagtgtatccaaatcatgagcagcatcttgtgaccctaggagcaaccatggcttaataacgccaacttgcaggtccgagctaaggtcctgcacataaccacaaccacccccactgctcggctctacttcttccacaacatgaattctggcatctttccatgtttctataattttctttccagttagcgttgtcaccctggtgcattgcttcctgagattattccgggagaatgctttaatttcctggttaagggagtacattacatgagcagtggctgggaacaaatacaaacaaatccagcaggcatagaaaacggctgaactgctagtcccttattgcccaggtaacaaagccagcctcagaggtgctcgcccatccaggtaaccgcagcagccacagaccaagagactgagtcgtccagctccgtttatcccagcgatgcaatgt

SEQ ID NO: 15390 - RNA, 4889 nt, Homo sapiens
  source 1..4889: mol_type = other RNA
gctgggattacaggcatgagccactgcgcctggccaccaacagattttttaattcagaatttgacagcaaataagtgttacatcttttaaaacaaatagcttcaaagaaatatattaatgggaaaatattaaacatatcatttttattaaagtatatcaacacctagaaacaataaagggtacatgatgaatatgtataaaaacaagtaactcaaagctttacttgaaatagaaaagtctaactataagttattttttgtgtgcatcaattgaaacaaaccataagtttgttgattataatgtcattttatgcattgcaagaatatacaacttcaaagtcttctggtttaaattcctaaataactacagggtaactaaatatgttcaggatccttcaggcagaaaaatcaactatttagagtcacctggaacaaataaataagtaatcatgccacatttctgttgtttttaaatttatcatggttttgcttataaaggtattgactcattaggttaactctgtaagattataagatgatattctgatttatacttgctacatttatgactacttggagaaacaacacttgaaggggaccttctatatacatttgaacaatctgagttacaaataatcatgctgacaaattcaggtttccccactaccactgaaattatcagagtctaagctgaaaaaaaaaaatccaagtattgtattcatacattttaatcaaggttcaatagggaagaagggaagaaaaagtaaaattgcaaacaaaatgttaaatactgtactccacttcctctgaaatatttgtcttttgaattagtatactggtctaaattttgcctccaaaaatctaagaagaatattgtttgggtttttcaaaaatctacatacttcttgagtgttctattcaaattttatgtaatcagaaacctattttaaggcataaaattagaaaaaaatttaaaaattattaacttcaattaacctcaaataaatagaattgtattgtatgctccactgcctttgttctactcagctttttcagtttgcggtttaaagcctccatatttcttttcaatgtttaaaaagacatgctgttttcattttccctttcctttaaaaaatggcagaataatctattgaaaaacaaagaggcaaaaactccttgaactatttttcctctcctttaaaacagacctatatttggtgtatgtatcttttaagtttgcagtatgtgagaaagaggaccgtaatcataaagttctttttttaaaataactaggaatgacagagtgatttatccccatgggaagtgcaataaacatattgtatagtatatatgaccttatgctttacttggtgcccctaaaagactgaattatattcattgatctattttaatacagcaaactacaatttaacgttaaaacaaatttgatgctcaaagcacttctgtagaagatacaaaagataaatgtttgaatcttacccagatcactataggcaacaactaagcatataaactacagacataaataatacacaatccaggccaggtgtagtggctaacaccgtaatcccagcactttgggagaccaaggcgtgtggatcacttgcggtcaggagttcgagaccagcctgaccaacatggttgaaccctgtctctaccaaaaaaaaatacaaaatttgctgggcatggtggcacatgcctataatcccagctacttgggaggctgatacaggagaatcgcttgaagctgggaggcagaggttgcagtgagccaagatcacgccactgcactccagcctgggcaataagagcaaaactctgtctcaaataataataatatcattaagagcaaaactccatctcaaaaataataataatacatgagccattatgaacaaattctatcaaggcttcatgtgacatttaatggctgaaaactaaacaggatttagcaaaataaaatgtatttaaatacatcctttcttatgaaaggagaaggcttatccagtgatactgaccatagagagaacctatacatcagtctcatatttaagagggttctgcctgccttggttggcttcaaagagctcactgtacgttgattatatttagactgcttcttagcagaagcaaagagtttataacagttcataacatcacaagtgatggcatcttgtcacggtgtaagcaatctcaaaacataacttgcatttatcacttctactttttgctcatgacagcatatgaaagcctgccttctcaaatgcacagatgtgttcaatatgcactttccatctatgcttgctctttataatgtatatttaagaagagctcaagacttttaaaaataaaacctacatggcaatgatatcttctaagtcatgaaaaactatgtggaaactatcaggccaggcgtggtggctgatgcctgtaatcctagcacttgggaggctaaggcgggaggatcacttaagcctaggagtttgagatcagcctgggcaacatggcaagactcctgtctctacaaaaataaaaataaaattagccagatgtggtggcgcacagctgtagtctcagctactcaggagactgaggtgggaggactgcttgagcccaggaggtagaggctgcagtgcgttgtgttcatgccactccactctagcctaggtgacagagcaagaccctgtctcgaaaaaaaaaaaaaagaaaagaaaaaagaaactgtcttaattaattaattttaagtataccatattctgaagaaaaaatcaaaatctttaagcaaatttataatgtacagagctcagttcttcaaatacggagacattaaagaaaaaagaacctattcaaaggccaaagataaaactgtaaatgattgtgggtctcctaaaagtatatttaaagtttcttacaaaaccataacccttctcccctaaaaaatatgttctctggtagaatactgaagtagaaaacagaccactaaacaatgatcttgcagtatcaaacattttctcaaaaaattatgacataggatcaaaaaaacagaatgctaggcacccaagataaaaagcacaaaatgtaagagaatagatcacctgttcaaagaaccaaagctcacaataacgtatgacagaacacctatacattaaaaaaaaaaagaaagaaatgccgataacagaattgaaaaaaacaaaatgaggtcggatgcagtggctcacgcctgtaatcccagtatttagagaggccaaggtgggtggatcacctgaggtcaggagttcgagactgcctggcctatgtggtgagactccatctctactaaaaacacaaaaattagctgggcatggtggcaggcacctataatcccagctatatgggaggctggggcaggagaatcgcttgaacccgggaggcagaggttgcagtgagctgagattgcgccattgcactccagcctgggtgacaagagccaaactccatctaaaaaaagaaaaaaaaagaagaagacaaaatgaaaagtgtatatttttcataagagaacataagaattttgtgaatattgtagccactgtgtaaatattgtataaaccttcagatactggttatctcttttgggagatttaaggtattcatttttaatcttaaaaagattctttaaaaagaaatatacttccctttgaaatagtaagttaagtagcatttcaagtttttctttcataaaaacagttgctggaacagaaaaataggcttcattaaatgattctctccatgctctaaatacacattttaaatttaaacctttttcttctacagaaagcaatgattactaacactttgttattttcccttagcaatttaaaaaagcatttaatcacacattataataacaaagagaaagtaatgacatttgaaatttacttatacagtaggtcaggacaatcaaattgacctccatttatgcataaaaaaggcaagagaaaaaagggagttttgctagtctactctccaaaaaagggaaaagatggctatagaagtcaattcagaaactacagttgtccattgtctgctacaatgcaactcatgaactgttctcctgtattctgtcacacttattgctttctttgccctcttgatatgtacgaagctgctccatgaagccagaatttggacatatggaaggtcttgcatttttcaccaaagaaaaagcactggtaaatgaggtttgttcagaattcatcaggaaacctattacaattgcagcagccctggaaacgcctgcattacaatgaacaagaaccactccatcttttctttttgcttcttcaataaattcaaaacattctggaaaataagacaggatgttggtttcaggcagatccaatatagaaatgctcttatatgtaaagtcactgaggaaagcattttcaactccatatgcaacattaagaatatgagtcacctaggagcaaccatggcttaataacgccaacttgcaggtccgagctaaggtcctgcacataaccacaaccacccccactgctcggctctacttcttccacaacatgaattctggcatctttccatgtttctataattttctttccagttagcgttgtcaccctggtgcattgcttcctgagattattccgggagaatgctttaatttcctggttaagggagtacattacatgagcagtggctgggaacaaatacaaacaaatccagcaggcatagaaaacggctgaactgctagtcccttattgcccaggtaacaaagccagcctcagaggtgctcgcccatccaggtaaccgcagcagccacagaccaagagactgagtcgtccagctccgtttatcccagcgatgcaatgt

SEQ ID NO: 15391 - RNA, 4936 nt, Homo sapiens
  source 1..4936: mol_type = other RNA
gctgggattacaggcatgagccactgcgcctggccaccaacagattttttaattcagaatttgacagcaaataagtgttacatcttttaaaacaaatagcttcaaagaaatatattaatgggaaaatattaaacatatcatttttattaaagtatatcaacacctagaaacaataaagggtacatgatgaatatgtataaaaacaagtaactcaaagctttacttgaaatagaaaagtctaactataagttattttttgtgtgcatcaattgaaacaaaccataagtttgttgattataatgtcattttatgcattgcaagaatatacaacttcaaagtcttctggtttaaattcctaaataactacagggtaactaaatatgttcaggatccttcaggcagaaaaatcaactatttagagtcacctggaacaaataaataagtaatcatgccacatttctgttgtttttaaatttatcatggttttgcttataaaggtattgactcattaggttaactctgtaagattataagatgatattctgatttatacttgctacatttatgactacttggagaaacaacacttgaaggggaccttctatatacatttgaacaatctgagttacaaataatcatgctgacaaattcaggtttccccactaccactgaaattatcagagtctaagctgaaaaaaaaaaatccaagtattgtattcatacattttaatcaaggttcaatagggaagaagggaagaaaaagtaaaattgcaaacaaaatgttaaatactgtactccacttcctctgaaatatttgtcttttgaattagtatactggtctaaattttgcctccaaaaatctaagaagaatattgtttgggtttttcaaaaatctacatacttcttgagtgttctattcaaattttatgtaatcagaaacctattttaaggcataaaattagaaaaaaatttaaaaattattaacttcaattaacctcaaataaatagaattgtattgtatgctccactgcctttgttctactcagctttttcagtttgcggtttaaagcctccatatttcttttcaatgtttaaaaagacatgctgttttcattttccctttcctttaaaaaatggcagaataatctattgaaaaacaaagaggcaaaaactccttgaactatttttcctctcctttaaaacagacctatatttggtgtatgtatcttttaagtttgcagtatgtgagaaagaggaccgtaatcataaagttctttttttaaaataactaggaatgacagagtgatttatccccatgggaagtgcaataaacatattgtatagtatatatgaccttatgctttacttggtgcccctaaaagactgaattatattcattgatctattttaatacagcaaactacaatttaacgttaaaacaaatttgatgctcaaagcacttctgtagaagatacaaaagataaatgtttgaatcttacccagatcactataggcaacaactaagcatataaactacagacataaataatacacaatccaggccaggtgtagtggctaacaccgtaatcccagcactttgggagaccaaggcgtgtggatcacttgcggtcaggagttcgagaccagcctgaccaacatggttgaaccctgtctctaccaaaaaaaaatacaaaatttgctgggcatggtggcacatgcctataatcccagctacttgggaggctgatacaggagaatcgcttgaagctgggaggcagaggttgcagtgagccaagatcacgccactgcactccagcctgggcaataagagcaaaactctgtctcaaataataataatatcattaagagcaaaactccatctcaaaaataataataatacatgagccattatgaacaaattctatcaaggcttcatgtgacatttaatggctgaaaactaaacaggatttagcaaaataaaatgtatttaaatacatcctttcttatgaaaggagaaggcttatccagtgatactgaccatagagagaacctatacatcagtctcatatttaagagggttctgcctgccttggttggcttcaaagagctcactgtacgttgattatatttagactgcttcttagcagaagcaaagagtttataacagttcataacatcacaagtgatggcatcttgtcacggtgtaagcaatctcaaaacataacttgcatttatcacttctactttttgctcatgacagcatatgaaagcctgccttctcaaatgcacagatgtgttcaatatgcactttccatctatgcttgctctttataatgtatatttaagaagagctcaagacttttaaaaataaaacctacatggcaatgatatcttctaagtcatgaaaaactatgtggaaactatcaggccaggcgtggtggctgatgcctgtaatcctagcacttgggaggctaaggcgggaggatcacttaagcctaggagtttgagatcagcctgggcaacatggcaagactcctgtctctacaaaaataaaaataaaattagccagatgtggtggcgcacagctgtagtctcagctactcaggagactgaggtgggaggactgcttgagcccaggaggtagaggctgcagtgcgttgtgttcatgccactccactctagcctaggtgacagagcaagaccctgtctcgaaaaaaaaaaaaaagaaaagaaaaaagaaactgtcttaattaattaattttaagtataccatattctgaagaaaaaatcaaaatctttaagcaaatttataatgtacagagctcagttcttcaaatacggagacattaaagaaaaaagaacctattcaaaggccaaagataaaactgtaaatgattgtgggtctcctaaaagtatatttaaagtttcttacaaaaccataacccttctcccctaaaaaatatgttctctggtagaatactgaagtagaaaacagaccactaaacaatgatcttgcagtatcaaacattttctcaaaaaattatgacataggatcaaaaaaacagaatgctaggcacccaagataaaaagcacaaaatgtaagagaatagatcacctgttcaaagaaccaaagctcacaataacgtatgacagaacacctatacattaaaaaaaaaaagaaagaaatgccgataacagaattgaaaaaaacaaaatgaggtcggatgcagtggctcacgcctgtaatcccagtatttagagaggccaaggtgggtggatcacctgaggtcaggagttcgagactgcctggcctatgtggtgagactccatctctactaaaaacacaaaaattagctgggcatggtggcaggcacctataatcccagctatatgggaggctggggcaggagaatcgcttgaacccgggaggcagaggttgcagtgagctgagattgcgccattgcactccagcctgggtgacaagagccaaactccatctaaaaaaagaaaaaaaaagaagaagacaaaatgaaaagtgtatatttttcataagagaacataagaattttgtgaatattgtagccactgtgtaaatattgtataaaccttcagatactggttatctcttttgggagatttaaggtattcatttttaatcttaaaaagattctttaaaaagaaatatacttccctttgaaatagtaagttaagtagcatttcaagtttttctttcataaaaacagttgctggaacagaaaaataggcttcattaaatgattctctccatgctctaaatacacattttaaatttaaacctttttcttctacagaaagcaatgattactaacactttgttattttcccttagcaatttaaaaaagcatttaatcacacattataataacaaagagaaagtaatgacatttgaaatttacttatacagtaggtcaggacaatcaaattgacctccatttatgcataaaaaaggcaagagaaaaaagggagttttgctagtctactctccaaaaaagggaaaagatggctatagaagtcaattcagaaactacagttgtccattgtctgctacaatgcaactcatgaactgttctcctgtattctgtcacacttattgctttctttgccctcttgatatgtacgaagctgctccatgaagccagaatttggacatatggaaggtcttgcatttttcaccaaagaaaaagcactggtaaatgaggtttgttcagaattcatcaggaaacctattacaattgcagcagccctggaaacgcctgcattacaatgaacaagaaccactccatcttttctttttgcttcttcaataaattcaaaacattctggaaaataagacaggatgttggtttcaggcagatccaatatagaaatgctcttatatgtaaagtcactgaggaaagcattttcaactccatatgcaacattaagaatatgagtcaccttattctttttcagtgtatccaaatcatgagcagcatcttgtgaccctaggagcaaccatggcttaataacgccaacttgcaggtccgagctaaggtcctgcacataaccacaaccacccccactgctcggctctacttcttccacaacatgaattctggcatctttccatgtttctataattttctttccagttagcgttgtcaccctggtgcattgcttcctgagattattccgggagaatgctttaatttcctggttaagggagtacattacatgagcagtggctgggaacaaatacaaacaaatccagcaggcatagaaaacggctgaactgctagtcccttattgcccaggtaacaaagccagcctcagaggtgctcgcccatccaggtaaccgcagcagccacagaccaagagactgagtcgtccagctccgtttatcccagcgatgcaatgt

SEQ ID NO: 15392 - RNA, 4818 nt, Homo sapiens
  source 1..4818: mol_type = other RNA
gctgggattacaggcatgagccactgcgcctggccaccaacagattttttaattcagaatttgacagcaaataagtgttacatcttttaaaacaaatagcttcaaagaaatatattaatgggaaaatattaaacatatcatttttattaaagtatatcaacacctagaaacaataaagggtacatgatgaatatgtataaaaacaagtaactcaaagctttacttgaaatagaaaagtctaactataagttattttttgtgtgcatcaattgaaacaaaccataagtttgttgattataatgtcattttatgcattgcaagaatatacaacttcaaagtcttctggtttaaattcctaaataactacagggtaactaaatatgttcaggatccttcaggcagaaaaatcaactatttagagtcacctggaacaaataaataagtaatcatgccacatttctgttgtttttaaatttatcatggttttgcttataaaggtattgactcattaggttaactctgtaagattataagatgatattctgatttatacttgctacatttatgactacttggagaaacaacacttgaaggggaccttctatatacatttgaacaatctgagttacaaataatcatgctgacaaattcaggtttccccactaccactgaaattatcagagtctaagctgaaaaaaaaaaatccaagtattgtattcatacattttaatcaaggttcaatagggaagaagggaagaaaaagtaaaattgcaaacaaaatgttaaatactgtactccacttcctctgaaatatttgtcttttgaattagtatactggtctaaattttgcctccaaaaatctaagaagaatattgtttgggtttttcaaaaatctacatacttcttgagtgttctattcaaattttatgtaatcagaaacctattttaaggcataaaattagaaaaaaatttaaaaattattaacttcaattaacctcaaataaatagaattgtattgtatgctccactgcctttgttctactcagctttttcagtttgcggtttaaagcctccatatttcttttcaatgtttaaaaagacatgctgttttcattttccctttcctttaaaaaatggcagaataatctattgaaaaacaaagaggcaaaaactccttgaactatttttcctctcctttaaaacagacctatatttggtgtatgtatcttttaagtttgcagtatgtgagaaagaggaccgtaatcataaagttctttttttaaaataactaggaatgacagagtgatttatccccatgggaagtgcaataaacatattgtatagtatatatgaccttatgctttacttggtgcccctaaaagactgaattatattcattgatctattttaatacagcaaactacaatttaacgttaaaacaaatttgatgctcaaagcacttctgtagaagatacaaaagataaatgtttgaatcttacccagatcactataggcaacaactaagcatataaactacagacataaataatacacaatccaggccaggtgtagtggctaacaccgtaatcccagcactttgggagaccaaggcgtgtggatcacttgcggtcaggagttcgagaccagcctgaccaacatggttgaaccctgtctctaccaaaaaaaaatacaaaatttgctgggcatggtggcacatgcctataatcccagctacttgggaggctgatacaggagaatcgcttgaagctgggaggcagaggttgcagtgagccaagatcacgccactgcactccagcctgggcaataagagcaaaactctgtctcaaataataataatatcattaagagcaaaactccatctcaaaaataataataatacatgagccattatgaacaaattctatcaaggcttcatgtgacatttaatggctgaaaactaaacaggatttagcaaaataaaatgtatttaaatacatcctttcttatgaaaggagaaggcttatccagtgatactgaccatagagagaacctatacatcagtctcatatttaagagggttctgcctgccttggttggcttcaaagagctcactgtacgttgattatatttagactgcttcttagcagaagcaaagagtttataacagttcataacatcacaagtgatggcatcttgtcacggtgtaagcaatctcaaaacataacttgcatttatcacttctactttttgctcatgacagcatatgaaagcctgccttctcaaatgcacagatgtgttcaatatgcactttccatctatgcttgctctttataatgtatatttaagaagagctcaagacttttaaaaataaaacctacatggcaatgatatcttctaagtcatgaaaaactatgtggaaactatcaggccaggcgtggtggctgatgcctgtaatcctagcacttgggaggctaaggcgggaggatcacttaagcctaggagtttgagatcagcctgggcaacatggcaagactcctgtctctacaaaaataaaaataaaattagccagatgtggtggcgcacagctgtagtctcagctactcaggagactgaggtgggaggactgcttgagcccaggaggtagaggctgcagtgcgttgtgttcatgccactccactctagcctaggtgacagagcaagaccctgtctcgaaaaaaaaaaaaaagaaaagaaaaaagaaactgtcttaattaattaattttaagtataccatattctgaagaaaaaatcaaaatctttaagcaaatttataatgtacagagctcagttcttcaaatacggagacattaaagaaaaaagaacctattcaaaggccaaagataaaactgtaaatgattgtgggtctcctaaaagtatatttaaagtttcttacaaaaccataacccttctcccctaaaaaatatgttctctggtagaatactgaagtagaaaacagaccactaaacaatgatcttgcagtatcaaacattttctcaaaaaattatgacataggatcaaaaaaacagaatgctaggcacccaagataaaaagcacaaaatgtaagagaatagatcacctgttcaaagaaccaaagctcacaataacgtatgacagaacacctatacattaaaaaaaaaaagaaagaaatgccgataacagaattgaaaaaaacaaaatgaggtcggatgcagtggctcacgcctgtaatcccagtatttagagaggccaaggtgggtggatcacctgaggtcaggagttcgagactgcctggcctatgtggtgagactccatctctactaaaaacacaaaaattagctgggcatggtggcaggcacctataatcccagctatatgggaggctggggcaggagaatcgcttgaacccgggaggcagaggttgcagtgagctgagattgcgccattgcactccagcctgggtgacaagagccaaactccatctaaaaaaagaaaaaaaaagaagaagacaaaatgaaaagtgtatatttttcataagagaacataagaattttgtgaatattgtagccactgtgtaaatattgtataaaccttcagatactggttatctcttttgggagatttaaggtattcatttttaatcttaaaaagattctttaaaaagaaatatacttccctttgaaatagtaagttaagtagcatttcaagtttttctttcataaaaacagttgctggaacagaaaaataggcttcattaaatgattctctccatgctctaaatacacattttaaatttaaacctttttcttctacagaaagcaatgattactaacactttgttattttcccttagcaatttaaaaaagcatttaatcacacattataataacaaagagaaagtaatgacatttgaaatttacttatacagtaggtcaggacaatcaaattgacctccatttatgcataaaaaaggcaagagaaaaaagggagttttgctagtctactctccaaaaaagggaaaagatggctatagaagtcaattcagaaactacagttgtccattgtctgctacaatgcaactcatgaactgttctcctgtattctgtcacacttattgctttctttgccctcttgatatgtacgaagctgctccatgaagccagaatttggacatatggaaggtcttgcatttttcaccaaagaaaaagcactggtaaatgaggtttgttcagaattcatcaggaaacctattacaattgcagcagccctggaaacgcctgcattacaatgaacaagaaccactccatcttttctttttgcttcttcaataaattcaaaacattcttattctttttcagtgtatccaaatcatgagcagcatcttgtgaccctaggagcaaccatggcttaataacgccaacttgcaggtccgagctaaggtcctgcacataaccacaaccacccccactgctcggctctacttcttccacaacatgaattctggcatctttccatgtttctataattttctttccagttagcgttgtcaccctggtgcattgcttcctgagattattccgggagaatgctttaatttcctggttaagggagtacattacatgagcagtggctgggaacaaatacaaacaaatccagcaggcatagaaaacggctgaactgctagtcccttattgcccaggtaacaaagccagcctcagaggtgctcgcccatccaggtaaccgcagcagccacagaccaagagactgagtcgtccagctccgtttatcccagcgatgcaatgt

SEQ ID NO: 15393 - RNA, 2171 nt, Homo sapiens
  source 1..2171: mol_type = other RNA
gctgggattacaggcatgagccactgcgcctggccaccctcatgctcttaaccacagctgttcccaccccaggaaaacacatggctagtcattcaataaacagcataagagatgctatggggtatctggtgctgggcagactgaggtgaagtccctgggtgcttgcggctgaccctctaaataggaggagacagacactgaaggctgcattactcccaaggtgatgacagccaggtagggggccaggggacaattctgtaactaagccagtctaccttcgtccagagatcaagagagcctccctggttaaataagacagcctccaggctgcacaaaacttccggcacaatgagcaagacagacatgcattgaacagtatcacataaatcacttctattgcttaaaaggtggatgcaccagctgcagtggctcatgcctgtcatctcagcagtttgggaggctgagatggaaagatcacttgaacccagaagtaggagaccagcctgggcaaacagtgagacctccatctccccccagcccagaaaaattagccagacatggtggcacacgcctgtagtcccagatactggggaggttgaggtgggaggatgccttgagcctaaggggttgagtctgcagtgagctgggactgcaccactgctcttagcctgggcaaccgagcaagaccctgtctcaaagaaaaaaggtggatgctgccaaaagctaggtgctgttgcaaccggggcacagggggaagacacaggtctctgaccccagtccccaagctcagttaacagcagaagttacttacctggcaggaaaaccaggcttccagcatgacccttgcctccctctgcccgctcccggtccccgtccacttctcgggcccttccgccacaatgaggtggccagggctgctcacaccgggcccagccgcagcctgttcccctccttcatgcggctcttggagtgatcgattctgccacgggaatggccaggataatttttgcttagcttcaaatacctcgttttcaggaattcctctgccagaaggttataaagcttcctctaaaatgtgggggaaagattaagcctgcttatggttaataatacactgtcccctgtccgtcaaattgcctgtctgctattgaaagttcactattagatacttatttaaacagcctcgcaaggcttctgaagaaagtgcagttatgcatttttcccctccttgctggcgcgaacgactatagataaacatcaattggctcctgcggatcacagtcacagtaaataaatttttcaggaagcttgagatccgcacaaaggctccgccaagctcccatttcacacaacatcaatgtttggcctccaagaaataaaagctctaaggtgtccatcgccagggcaaaattatcaattgtcaagtcacttttaaaagaaaaagaagatagagggtttcagggagccatttcatcctgcagcttaaaataaaaggaagagcgacaggcgcttcacccacaaactaaccactgggacttccccctaaaagctcaggtgttcatcgcccccccgtcaaatttctggccccagccctgctgccctgggtgagctgaagcagtcagttcagcttggagctgccggttccagctgagttcagtgacttcagtgactcaggcgttgggttatttttactttctcaaagtgggtttttttttttcactacttttagaagtggcagacgaggcttgtctattataaaatatttgttgcaaacacgcacttacttgctcaccgccccacacacagttctcgtctgtgtaaaaatctcaagtcgccgtggtgtgaggggcaggagatgcaaaagctaggacaccctcctgggcgagccagagtttatgtaacagcacagttctactggagtcggggtcatctaagctgggaacctgaaacaggtgtcattttccagatagggaaactgaggtacaggggagccagaggaagtgagacatagaggtggatgtacctgcatttgcatctcagctccactacgttccaactgcatggccttgggcaggaaacttaaatctgttgggcctggcctggtgcagtggctcatgcttgcagtcccagcactttgggaggccaaggcaggtggatctcttgagcccagg

SEQ ID NO: 15394 - RNA, 3212 nt, Homo sapiens
  source 1..3212: mol_type = other RNA
gctgggattacaggcatgagccactgcgcctggccatgagataaactcatcctggggtctacactcaatgtccagattcaacagagagctcctggctggcccatgagccgtgtcaacttctaacacagcattcggtatctcacagtgtgacttttttccttgatccaaccatgaagacatctcagtctctccacaactattcaagactcacacttgaaattctaaggtttccttgatgtttaaagagagtctgtttattgctatttctaacttctattgcatagatctgtgcaatgctgaaatttagggtacttttctctcctctgctataatctggagtagccttacaaaatctgagttgtagctacctggtgcggcactcatagagagtggggcatgaaatcttccctctctctttgcattgctggtttgcattattgggggtattagatgaccctggcttttggcaagaggagtctagatggaggtttggtgctaactgacacagtttcttgcagcagatagaaataatcaaacctggttttctctgtgttagtatctcacacacacttccactccaaatacatccctgatgctgattaacctttgtgtttataattgtatgtcgtctacaaggtcccttgtaaaccttaaagcatgacaaatagaggttactatatgttcatggattgtctttcttttaggggggaagggatagggtctcactctgtcatccatgctagactgcagtggcacagtcatagttcactgtaagctcaaacttctggacttaggcagtaatcccagttcagtctcccaggtagctgggactacaggcatgtaccaccatgccaagctatttttttctaagtttttgtagatatgcagtcttgctatgttgtcaagtctagtcttgaactcctggcctcaagcaatcctcctgccttggcatcccaaggtgctggaattataagtgtgagccacagtgcttggctggaacgtaattttctttttttctttctttctttcttctttgagacagtctcactctgtcgcccaggctggagtgcagtggtgtgatctcagctcactgcaacctccacctaccgggtcaagcgattcttatgcctcagcctcccaagtagctagggttacaggcatgtgccaacatgcctggctaatttttgtatttttagtagagatggggtttcgccatgttagccatgctggtctcaaactcctgacctcaggtgatccgcctgcctcggcctcccaaagtgctgggattacaggcatgagtcaccacggaacgtaatttttaacaatagccttcggtaatccaatttagttgttcccagtgaatttctcctacatcattacatttttttctgggtagagtttactgaagaaggtcttcttcatggcgaccttcagctccttgttcctgaggctgaagatgatggggctgaggaagggtgtgaggaccgtgtaggtgatgcccatcaaggtgtctccttccagagactggggacttttgggcttcaggtaaatgacggaggcaaagccatagtgcacgaccaccacagtgaggtgagaggcacaggtggagaaggccttgttccgaccttcagcagaagggatcttcaagatggcggccacgatgaaggcataggagaggaggatgaggagaaaacagcccagcagggccgtgatacacaccaagcccacgcctttggccaccaccagcacatcgtctccacaggccaacttcaacagaggtggcacatggcaagcaaaatggtggatctccttgtgtccacagaaggcgaggtggaaaatggccgaggtcaccaccatccccatgaccaagccaccagcccaggagcagcccaccaggcaggcgcagccccgcgggctcatgagcacgttgtagcgcagggggtggcagatggccacgtagcggtcgtagcccatgacggtgagcaggaaggagtgggtgaagccgaagctgaaggagaagaacatctgactggcacaggccaggaaggcgatggagcgctgggtggacagcaggtcggccagcatgcgcgggatgatggccacggtgtagaggatctcggagacggagagggcgcacaggaagaggtacatgggcgtgtggaggctgcgctcgctccagacggtggccatgatgagcaggttgcccagcagcgtgaacaggtacatcagcaggaacagcaggaagagcatcagctggaggtgggggaagacagagaagccgacgaggatgaattgggtcactgtggagtgattggctctctgcatggaggctgtgcctgtagtcccagctcttcgggaggcagagacaggagaatctcttgaacctgggaggcggaggttgcagtaagccgagatggcgccactggactccaccctggcgacagagcgagtctcagttgctggtggctgtttcaaaggccactaggagatgctgcttccccatgactgaccgtctacacactcttgttcatatcaattcagatcacaagaatcgacagcgagtgagtgaacaaggtggggggagagagagagagagaaaaggaggaggaggaggaggaggaaaagaaagaaaaaagggaggaagaaagagagggagggagggaggaaggaaagaaggataaaaggaaggaaggatggggactgcaggaggaaggaaggagggagggagggaaggaggaaggaaggaacgaaggaaggaaggaaggagagtgagggaggaaaggaggagagtgaggaaggaagaaaggagggagggaggcaggaaggaaggagagtgagggaggaaagaaggagagtgaggaaggaaggaagaaagggagggagggaggcaggaaggaaggaaggagagtgagggaggaaagaaggagagtgagataggaagaaacgagggagggaggaatggagggaggaaggaagggagggagggagaaaccttgagaggacaggagccgatcacgtctgtaggaggtagctgagggctgcatgtaacaccgtctggaatgatgggatgcagaatgcagctaaaagggtagtccagtcattctgggactccaggcatctgcttctgcttcatcccagtaggaggctctagtttggagtttctccacaggtgggagctgaccaggtgtgggctgcaccaagcagccacacca

SEQ ID NO: 15395 - RNA, 1379 nt, Homo sapiens
  source 1..1379: mol_type = other RNA
gctgggattacaggcatgagccactgcgcctggccatgttttagtaactttgatggttacttattcaaaactagcagagtgtccctgaagtttggtaaaaaaaaaaaagtagttctcaaaaattagtgtctaaaagccaccagaaatcagagaacaggagaccatttgattaatctaaatttaaattcgagtcatcatgtagctgaattcttgggactatggtaaatttctgattgtctcctctatgtgagttttttaaaaataaaagaaaaaagccaatagtgattgtctagaataacttttaaaatgtaaaaacccgggcatgttctttgtaaagtgttcatgcatttccaaagtggataagaaacaggatttatgggactggaagtgccacagagtgtggagaggcttcttgacatagtgtggccacctgagaagagcaatgaggggacctgacacctggagaaagagcagccaagagacccaagaggagcaggcgagaggctcagggaaaagcaggggcgccatctccctgccactcccttggggggccctgcctacactgtcaccatgatctggtccagaggtttgcgcttgaggtcaggcaccgtggcctccttgctggggtaccccacggggagcagcatcagcagcttttcatgtgcggggcggcccaggagcaccctcagtcgagggccacagttgagaggagtggtagtgacagtcaccagacctgcattctgcagggcagctagcaggatgccacaagcgatggaaacactgatctcattgtagtagtggacttttttcttgccatttgcggcgaaaccatgtacttgtttgaaaatgagaatcaaaataggggcagtatccaagtactctttaatccagttggttctcagtttcttgaggtctgtgacccagcgatgtcccatccttttcatgtagttgatctcctcttcctcctcaatgatctttcgaatcttgtgcttcacgtctgggtccttcacaaccacgaaggtccagggctctgtgtgagccccactcggggctgttccgtctcttattgagaagttcataaaattcctgagacctcttaaccatttccttctcaggatagtggttatgagagaaggggatgtgttcaacattttcttctgattcttgccattcatcagcatcttcttctgcttggtgcaggtcactgctgtcttttaagtcttcatccacccaggggcgagcttcggccctggttctaggctcccccttctttttctccatgcttctgtcggcatttttaaagatccacacaaccaaaatgcagagaatggctaccaagatgggagtcaggaaatacatggtctggagtctgacgtcac

SEQ ID NO: 15396 - RNA, 1447 nt, Homo sapiens
  source 1..1447: mol_type = other RNA
gctgggattacaggcatgagccactgcgcctggccatgttttagtaactttgatggttacttattcaaaactagcagagtgtccctgaagtttggtaaaaaaaaaaaagtagttctcaaaaattagtgtctaaaagccaccagaaatcagagaacaggagaccatttgattaatctaaatttaaattcgagtcatcatgtagctgaattcttgggactatggtaaatttctgattgtctcctctatgtgagttttttaaaaataaaagaaaaaagccaatagtgattgtctagaataacttttaaaatgtaaaaacccgggcatgttctttgtaaagtgttcatgcatttccaaagtggataagaaacaggatttatgggactggaagtgccacagagtgtggagaggcttcttgacatagtgtggccacctgagaagagcaatgaggggacctgacacctggagaaagagcagccaagagacccaagaggagcaggcgagaggctcagggaaaagcaggggcgccatctccctgccactcccttggggggccctgcctacactgtcaccatgatctggtccagaggtttgcgcttgaggtcaggcaccgtggcctccttgctggggtaccccacggggagcagcatcagcagcttttcatgtgcggggcggcccaggagcaccctcagtcgagggccacagttgagaggagtggtagtgacagtcaccagacctgcattctgcagggcagctagcaggatgccacaagcgatggaaacactgatctcattgtagtagtggacttttttcttgccatttgcggcgaaaccatgtacttgtttgaaaatgagaatcaaaataggggcagtatccaagtactctttaatccagttggttctcagtttcttgaggtctgtgacccagcgatgtcccatccttttcatgtagttgatctcctcttcctcctcaatgatctttcgaatcttgtgcttcacgtctgggtccttcacaaccacgaaggtccagggctctgtgtgagccccactcggggctgttcctgccgttctgatgacattatcaatgacttccattgggacttgctcattacttatgaacctgactgaccgtctcttattgagaagttcataaaattcctgagacctcttaaccatttccttctcaggatagtggttatgagagaaggggatgtgttcaacattttcttctgattcttgccattcatcagcatcttcttctgcttggtgcaggtcactgctgtcttttaagtcttcatccacccaggggcgagcttcggccctggttctaggctcccccttctttttctccatgcttctgtcggcatttttaaagatccacacaaccaaaatgcagagaatggctaccaagatgggagtcaggaaatacatggtctggagtctgacgtcac

SEQ ID NO: 15397 - RNA, 1508 nt, Homo sapiens
  source 1..1508: mol_type = other RNA
gctgggattacaggcatgagccactgcgcctggccatgttttagtaactttgatggttacttattcaaaactagcagagtgtccctgaagtttggtaaaaaaaaaaaagtagttctcaaaaattagtgtctaaaagccaccagaaatcagagaacaggagaccatttgattaatctaaatttaaattcgagtcatcatgtagctgaattcttgggactatggtaaatttctgattgtctcctctatgtgagttttttaaaaataaaagaaaaaagccaatagtgattgtctagaataacttttaaaatgtaaaaacccgggcatgttctttgtaaagtgttcatgcatttccaaagtggataagaaacaggatttatgggactggaagtgccacagagtgtggagaggcttcttgacatagtgtggccacctgagaagagcaatgaggggacctgacacctggagaaagagcagccaagagacccaagaggagcaggcgagaggctcagggaaaagcaggggcgccatctccctgccactcccttggggggccctgcctacactgtcaccatgatctggtccagaggtttgcgcttgaggtcaggcaccgtggcctccttgctggggtaccccacggggagcagcatcagcagcttttcatgtgcggggcggcccaggagcaccctcagtcgagggccacagttgagaggagtggtagtgacagtcaccagacctgcattctgcttacagattcaggaaggaaatcaatgccagctccttcaggataatttttccaaaaacctgcagggcagctagcaggatgccacaagcgatggaaacactgatctcattgtagtagtggacttttttcttgccatttgcggcgaaaccatgtacttgtttgaaaatgagaatcaaaataggggcagtatccaagtactctttaatccagttggttctcagtttcttgaggtctgtgacccagcgatgtcccatccttttcatgtagttgatctcctcttcctcctcaatgatctttcgaatcttgtgcttcacgtctgggtccttcacaaccacgaaggtccagggctctgtgtgagccccactcggggctgttcctgccgttctgatgacattatcaatgacttccattgggacttgctcattacttatgaacctgactgaccgtctcttattgagaagttcataaaattcctgagacctcttaaccatttccttctcaggatagtggttatgagagaaggggatgtgttcaacattttcttctgattcttgccattcatcagcatcttcttctgcttggtgcaggtcactgctgtcttttaagtcttcatccacccaggggcgagcttcggccctggttctaggctcccccttctttttctccatgcttctgtcggcatttttaaagatccacacaaccaaaatgcagagaatggctaccaagatgggagtcaggaaatacatggtctggagtctgacgtcac

SEQ ID NO: 15398 - RNA, 1559 nt, Homo sapiens
  source 1..1559: mol_type = other RNA
gctgggattacaggcatgagccactgcgcctggccatgttttagtaactttgatggttacttattcaaaactagcagagtgtccctgaagtttggtaaaaaaaaaaaagtagttctcaaaaattagtgtctaaaagccaccagaaatcagagaacaggagaccatttgattaatctaaatttaaattcgagtcatcatgtagctgaattcttgggactatggtaaatttctgattgtctcctctatgtgagttttttaaaaataaaagaaaaaagccaatagtgattgtctagaataacttttaaaatgtaaaaacccgggcatgttctttgtaaagtgttcatgcatttccaaagtggataagaaacaggatttatgggactggaagtgccacagagtgtggagaggcttcttgacatagtgtggccacctgagaagagcaatgaggggacctgacacctggagaaagagcagccaagagacccaagaggagcaggcgagaggctcagggaaaagcaggggcgccatctccctgccactcccttggggggccctgcctacactgtcaccatgatctggtccagaggtttgcgcttgaggtcaggcaccgtggcctccttgctggggtaccccacggggagcagcatcagcagcttttcatgtgcggggcggcccaggagcaccctcagtcgagggccacagttgagaggagtggtagtgacagtcaccagacctgcattctgggcagccttgtgagctgagcttgctgcaggcttcgctgcttcttccaggaccctcaatcaggtggcggtgcctcgcagtctgatgccgcatggtgattccattatttacctgcagggcagctagcaggatgccacaagcgatggaaacactgatctcattgtagtagtggacttttttcttgccatttgcggcgaaaccatgtacttgtttgaaaatgagaatcaaaataggggcagtatccaagtactctttaatccagttggttctcagtttcttgaggtctgtgacccagcgatgtcccatccttttcatgtagttgatctcctcttcctcctcaatgatctttcgaatcttgtgcttcacgtctgggtccttcacaaccacgaaggtccagggctctgtgtgagccccactcggggctgttcctgccgttctgatgacattatcaatgacttccattgggacttgctcattacttatgaacctgactgaccgtctcttattgagaagttcataaaattcctgagacctcttaaccatttccttctcaggatagtggttatgagagaaggggatgtgttcaacattttcttctgattcttgccattcatcagcatcttcttctgcttggtgcaggtcactgctgtcttttaagtcttcatccacccaggggcgagcttcggccctggttctaggctcccccttctttttctccatgcttctgtcggcatttttaaagatccacacaaccaaaatgcagagaatggctaccaagatgggagtcaggaaatacatggtctggagtctgacgtcac

SEQ ID NO: 15399 - RNA, 1620 nt, Homo sapiens
  source 1..1620: mol_type = other RNA
gctgggattacaggcatgagccactgcgcctggccatgttttagtaactttgatggttacttattcaaaactagcagagtgtccctgaagtttggtaaaaaaaaaaaagtagttctcaaaaattagtgtctaaaagccaccagaaatcagagaacaggagaccatttgattaatctaaatttaaattcgagtcatcatgtagctgaattcttgggactatggtaaatttctgattgtctcctctatgtgagttttttaaaaataaaagaaaaaagccaatagtgattgtctagaataacttttaaaatgtaaaaacccgggcatgttctttgtaaagtgttcatgcatttccaaagtggataagaaacaggatttatgggactggaagtgccacagagtgtggagaggcttcttgacatagtgtggccacctgagaagagcaatgaggggacctgacacctggagaaagagcagccaagagacccaagaggagcaggcgagaggctcagggaaaagcaggggcgccatctccctgccactcccttggggggccctgcctacactgtcaccatgatctggtccagaggtttgcgcttgaggtcaggcaccgtggcctccttgctggggtaccccacggggagcagcatcagcagcttttcatgtgcggggcggcccaggagcaccctcagtcgagggccacagttgagaggagtggtagtgacagtcaccagacctgcattctgggcagccttgtgagctgagcttgctgcaggcttcgctgcttcttccaggaccctcaatcaggtggcggtgcctcgcagtctgatgccgcatggtgattccattatttacctgcttacagattcaggaaggaaatcaatgccagctccttcaggataatttttccaaaaacctgcagggcagctagcaggatgccacaagcgatggaaacactgatctcattgtagtagtggacttttttcttgccatttgcggcgaaaccatgtacttgtttgaaaatgagaatcaaaataggggcagtatccaagtactctttaatccagttggttctcagtttcttgaggtctgtgacccagcgatgtcccatccttttcatgtagttgatctcctcttcctcctcaatgatctttcgaatcttgtgcttcacgtctgggtccttcacaaccacgaaggtccagggctctgtgtgagccccactcggggctgttcctgccgttctgatgacattatcaatgacttccattgggacttgctcattacttatgaacctgactgaccgtctcttattgagaagttcataaaattcctgagacctcttaaccatttccttctcaggatagtggttatgagagaaggggatgtgttcaacattttcttctgattcttgccattcatcagcatcttcttctgcttggtgcaggtcactgctgtcttttaagtcttcatccacccaggggcgagcttcggccctggttctaggctcccccttctttttctccatgcttctgtcggcatttttaaagatccacacaaccaaaatgcagagaatggctaccaagatgggagtcaggaaatacatggtctggagtctgacgtcac

SEQ ID NO: 15400 - RNA, 2447 nt, Homo sapiens
  source 1..2447: mol_type = other RNA
gctgggattacaggcatgagccactgcgcctggcccaatttatttttttttgtagtttcattctcctcacatccaaacagctacagcttccctccttttgtggggtccccaaaccaagtctcttttcaggagagcagacatgtgcctccacacagttctgaagttctgggggctccacattgtcagctgggttggggtctcccatgtgagggaggctgatggcactcgcaggtttttgcctcatctatgtacaaaggctcagaaaatttcttcggcatttgggaccctcgtgttctgtagctccaccagtcgctgcacagcctcaggcaagtcccactccccaaggcgacgattatctcgagtccgaatgttcactgttctcttactttgctctttctggccaaccacaaactgaaaattgtagtgggcaagctgggcccggcggattctccggctgagggtcagtccagagtctgcatccaggtcactgaccagtcctgcagcccgcaggctctgctgtgcctctttggcgtattcctcttgctcactccccacagggatgaccaccacctggaacggggacagccacagtggccatttccccccgcagctttctgccagcactcccaacagtctttccacagaaccgagcactgctcggtgaatgaggactggacgctccagggcacccgcctgccccttatactggaggtcaaatctcaggggcagttggaagtcaagctgaattgtcccacactgatgtggccggcccagggcatcgtggaggtgcacgtcaatcttaggtccatagaaggcaccatctccagagttgaggtcccagggttctccaaattccttcagggcctgtttaaggacctgttcggcctggtcccaaaggcaagggtcccccaggaagccagatggccgggtggacagtgccaggcggaaggagaagccaagaacggcatagacggaacggaggaaatcaagacagctttggatctctgcttccagctgatctgttgtacagaagatgtgagcgtcatcctgctggaagcaccgcagtcgggtcagtccccccagaccaccagaggcttcggcccggtgtagagccccaaagtcagctagtcgcaggggcagttcccgccaggatctgggccggtgggcgaacatcaggcagtgtgcagggcagttcataggcttgagggcgagtgtatctgtgatatgcctggtagaatcgtcactctgggagctgggaggcctgtcagagcctgggggctgcacggcaaacatgtcttcctgataatgctcccagtgccctgactgttcccagagcttcgtagaaaacagtgtgggagttttcacctcggagaaaccacgatgggcatactcagccctgataaacgccactagtgcattatacacccttgtccctcgtggcaggaagaagcagctcccagggctcagttcatggaagaagaagagctcctgttccttcccaatgcgccggtggtcccgcaattctgcttcctccctccatgcttcccagaccctcagcaattctgttgtggggaaggaaatccctgacactctctgcagtgtctctggggcccctgaagacctccataaggatgatgagttcgatagcagcttcagtcctccaatctgtccagtatgccgaaggtgggggccctggcaaaggtcaaccaatgtgccacacccatatactgttgctgttggacctgtcactttctcctcaatcaagtgaagcttaaaggggttatccttgaacaactggcgaagctgatcccgtgaagcctctagcctccggaagggtcgagcagcagctgtaagttcctggcaaatccgctccaaaacaggcagctctgagccccggattgtcctctcctttcccaggaagaaatcatggtaaaagccatattctgtacttggacctctgcagagaacagcacctaggaattgttcagctgctgcccccaggacatgggtgctggagtgccagaacactgctttcccctctggggaatcgaatgtcagaaatctgaggtcagaatctgtctccaagggccgctccagatcataaggttctccattcacttgagcagccactgcagtatctgccagtgttgaactgatctgccgggctagttggtagggggttgtgttccatgccacagcatcaattttctggcctccaggaagtgatatcttaatagtccggggttccttctgtgccatgcttgctaatctctttacctgagcagcccacagctcctcaaaaaggccaagccgctctgccaaccagcgtggaggggtcgacacaactgccgtgtgtagcctgcaagcctgtaaaccttggagccggagacaccgccacctctgatacagggccatgttccttcacaccagtgcctacatcctcaaac

SEQ ID NO: 15401 - RNA, 2322 nt, Homo sapiens
  source 1..2322: mol_type = other RNA
gctgggattacaggcatgagccactgcgcctggcccaatttatttttttttgtagtttcattctcctcacatccaaacagctacagcttccctccttttgtggggtccccaaaccaagtctcttttcaggagagcagacatgtgcctccacacagttctgaagttctgggggctccacattgtcagctgggttggggtctcccatgtgagggaggctgatggcactcgcaggtttttgcctcatctatgtacaaaggctcagaaaatttcttcggcatttgggaccctcgtgttctgtagctccaccagtcgctgcacagcctcaggcaagtcccactccccaaggcgacgattatctcgagtccgaatgttcactgttctcttactttgctctttctggccaaccacaaactgaaaattgtagtgggcaagctgggcccggcggattctccggctgagggtcagtccagagtctgcatccaggtcactgaccagtcctgcagcccgcaggctctgctgtgcctctttggcgtattcctcttgctcactccccacagggatgaccaccacctggaacggggacagccacagtggccatttccccccgcagctttctgccagcactcccaacagtctttccacagaaccgagcactgctcggtgaatgaggactggacgctccagggcacccgcctgccccttatactggaggtcaaatctcaggggcagttggaagtcaagctgaattgtcccacactgatgtggccggcccagggcatcgtggaggtgcacgtcaatcttaggtccatagaaggcaccatctccagagttgaggtcccagggttctccaaattccttcagggcctgtttaaggacctgttcggcctggtcccaaaggcaagggtcccccaggaagccagatggccgggtggacagtgccaggcggaaggagaagccaagaacggcatagacggaacggaggaaatcaagacagctttggatctctgcttccagctgatctgttgtacagaagatgtgagcgtcatcctgctggaagcaccgcagtcgggtcagtccccccagaccaccagaggcttcggcccggtgtagagccccaaagtcagctagtcgcaggggcagttcccgccaggatctgggccggtgggcgaacatcaggcagtgtgcagggcagttcataggcttgagggcgagtgtatctgtgatatgcctggtagaatcgtcactctgggagctgggaggcctgtcagagcctgggggctgcacggcaaacatgtcttcctgataatgctcccagtgccctgactgttcccagagcttcgtagaaaacagtgtgggagttttcacctcggagaaaccacgatgggcatactcagccctgataaacgccactagtgcattatacacccttgtccctcgtggcaggaagaagcagctcccagggctcagttcatggaagaagaagagctcctgttccttcccaatgcgccggtggtcccgcaattctgcttcctccctccatgcttcccagaccctcagcaattctgttgtggggaaggaaatccctgacactctctgcagtgtctctggggcccctgaagacctccataaggatgatgagttcgatagcagcttcagtcctccaatctgtccagtatgccgaaggtgggggccctggcaaaggtcaaccaatgtgccacacccatatactgttgctgttggacctgtcactttctcctcaatcaagtgaagcttaaaggggttatccttgaacaactggcgaagctgatcccgtgaagcctctagcctccggaagggtcgagcagcagctgtaagttcctggcaaatccgctccaaaacaggcagctctgagccccggattgtctgctttcccctctggggaatcgaatgtcagaaatctgaggtcagaatctgtctccaagggccgctccagatcataaggttctccattcacttgagcagccactgcagtatctgccagtgttgaactgatctgccgggctagttggtagggggttgtgttccatgccacagcatcaattttctggcctccaggaagtgatatcttaatagtccggggttccttctgtgccatgcttgctaatctctttacctgagcagcccacagctcctcaaaaaggccaagccgctctgccaaccagcgtggaggggtcgacacaactgccgtgtgtagcctgcaagcctgtaaaccttggagccggagacaccgccacctctgatacagggccatgttccttcacaccagtgcctacatcctcaaac

SEQ ID NO: 15402 - RNA, 2201 nt, Homo sapiens
  source 1..2201: mol_type = other RNA
gctgggattacaggcatgagccactgcgcctggcccaatttatttttttttgtagtttcattctcctcacatccaaacagctacagcttccctccttttgtggggtccccaaaccaagtctcttttcaggagagcagacatgtgcctccacacagttctgaagttctgggggctccacattgtcagctgggttggggtctcccatgtgagggaggctgatggcactcgcaggtttttgcctcatctatgtacaaaggctcagaaaatttcttcggcatttgggaccctcgtgttctgtagctccaccagtcgctgcacagcctcaggcaagtcccactccccaaggcgacgattatctcgagtccgaatgttcactgttctcttactttgctctttctggccaaccacaaactgaaaattgtagtgggcaagctgggcccggcggattctccggctgagggtcagtccagagtctgcatccaggtcactgaccagtcctgcagcccgcaggctctgctgtgcctctttggcgtattcctcttgctcactccccacagggatgaccaccacctggaacggggacagccacagtggccatttccccccgcagctttctgccagcactcccaacagtctttccacagaaccgagcactgctcggtgaatgaggactggacgctccagggcacccgcctgccccttatactggaggtcaaatctcaggggcagttggaagtcaagctgaattgtcccacactgatgtggccggcccagggcatcgtggaggtgcacgtcaatcttaggtccatagaaggcaccatctccagagttgaggtcccagggttctccaaattccttcagggcctgtttaaggacctgttcggcctggtcccaaaggcaagggtcccccaggaagccagatggccgggtggacagtgccaggcggaaggagaagccaagaacggcatagacggaacggaggaaatcaagacagctttggatctctgcttccagctgatctgttgtacagaagatgtgagcgtcatcctgctggaagcaccgcagtcgggtcagtccccccagaccaccagaggcttcggcccggtgtagagccccaaagtcagctagtcgcaggggcagttcccgccaggatctgggccggtgggcgaacatcaggcagtgtgcagggcagttcataggcttgagggcgagtgtatctgtgatatgcctggtagaatcgtcactctgggagctgggaggcctgtcagagcctgggggctgcacggcaaacatgtcttcctgataatgctcccagtgccctgactgttcccagagcttcgtagaaaacagtgtgggagttttcacctcggagaaaccacgatgggcatactcagccgatagcagcttcagtcctccaatctgtccagtatgccgaaggtgggggccctggcaaaggtcaaccaatgtgccacacccatatactgttgctgttggacctgtcactttctcctcaatcaagtgaagcttaaaggggttatccttgaacaactggcgaagctgatcccgtgaagcctctagcctccggaagggtcgagcagcagctgtaagttcctggcaaatccgctccaaaacaggcagctctgagccccggattgtcctctcctttcccaggaagaaatcatggtaaaagccatattctgtacttggacctctgcagagaacagcacctaggaattgttcagctgctgcccccaggacatgggtgctggagtgccagaacactgctttcccctctggggaatcgaatgtcagaaatctgaggtcagaatctgtctccaagggccgctccagatcataaggttctccattcacttgagcagccactgcagtatctgccagtgttgaactgatctgccgggctagttggtagggggttgtgttccatgccacagcatcaattttctggcctccaggaagtgatatcttaatagtccggggttccttctgtgccatgcttgctaatctctttacctgagcagcccacagctcctcaaaaaggccaagccgctctgccaaccagcgtggaggggtcgacacaactgccgtgtgtagcctgcaagcctgtaaaccttggagccggagacaccgccacctctgatacagggccatgttccttcacaccagtgcctacatcctcaaac

SEQ ID NO: 15403 - RNA, 1846 nt, Homo sapiens
  source 1..1846: mol_type = other RNA
gctgggattacaggcatgagccactgcgcctggcccaatttatttttttttgtagtttcattctcctcacatccaaacagctacagcttccctccttttgtggggtccccaaaccaagtctcttttcaggagagcagacatgtgcctccacacagttctgaagttctgggggctccacattgtcagctgggttggggtctcccatgtgagggaggctgatggcactcgcaggtttttgcctcatctatgtacaaaggctcagaaaatttcttcggcatttgggaccctcgtgttctgtagctccaccagtcgctgcacagcctcaggcaagtcccactccccaaggcgacgattatctcgagtccgaatgttcactgttctcttactttgctctttctggccaaccacaaactgaaaattgtagtgggcaagctgggcccggcggattctccggctgagggtcagtccagagtctgcatccaggtcactgaccagtcctgcagcccgcaggctctgctgtgcctctttggcgtattcctcttgctcactccccacagggatgaccaccacctggaacggggacagccacagtggccatttccccccgcagctttctgccagcactcccaacagtctttccacagaaccgagcactgctcggtgaatgaggactggacgctccagggcacccgcctgccccttatactggaggtcaaatctcaggggcagttggaagtcaagctgaattgtcccacactgatgtggccggcccagggcatcgtggaggtgcacgtcaatcttaggtccatagaaggcaccatctccagagttgaggtcccagggttctccaaattccttcagggcctgtttaaggacctgttcggcctggtcccaaaggcaagggtcccccaggaagccagatggccgggtggacagtgccaggcggaaggagaagccaagaacggcatagacggaacggaggaaatcaagacagctttggatctctgcttccagctgatctgttgtacagaagatgtgagcgtcatcctgctggaagcaccgcagtcgggtcagtccccccagaccaccagaggcttcggcccggtgtagagccccaaagtcagctagtcgcaggggcagttcccgccaggatctgggccggtgggcgaacatcaggcagtgtgcagggcagttcataggcttgagggcgagtgtatctgtgatatgcctggtagaatcgtcactctgggagctgggaggcctgtcagagcctgggggctgcacggcaaacatgtcttcctgataatgctcccagtgccctgactgttcccagagcttcgtagaaaacagtgtgggagttttcacctcggagaaaccacgatgggcatactcagccgatagcagcttcagtcctccaatctgtccagtatgccgaaggtgggggccctggcaaaggtcaaccaatgtgccacacctctcctttcccaggaagaaatcatggtaaaagccatattctgtacttggaccactgcagtatctgccagtgttgaactgatctgccgggctagttggtagggggttgtgttccatgccacagcatcaattttctggcctccaggaagtgatatcttaatagtccggggttccttctgtgccatgcttgctaatctctttacctgagcagcccacagctcctcaaaaaggccaagccgctctgccaaccagcgtggaggggtcgacacaactgccgtgtgtagcctgcaagcctgtaaaccttggagccggagacaccgccacctctgatacagggccatgttccttcacaccagtgcctacatcctcaaac

SEQ ID NO: 15404 - RNA, 2057 nt, Homo sapiens
  source 1..2057: mol_type = other RNA
gctgggattacaggcatgagccactgcgcctggcccaatttatttttttttgtagtttcattctcctcacatccaaacagctacagcttccctccttttgtggggtccccaaaccaagtctcttttcaggagagcagacatgtgcctccacacagttctgaagttctgggggctccacattgtcagctgggttggggtctcccatgtgagggaggctgatggcactcgcaggtttttgcctcatctatgtacaaaggctcagaaaatttcttcggcatttgggaccctcgtgttctgtagctccaccagtcgctgcacagcctcaggcaagtcccactccccaaggcgacgattatctcgagtccgaatgttcactgttctcttactttgctctttctggccaaccacaaactgaaaattgtagtgggcaagctgggcccggcggattctccggctgagggtcagtccagagtctgcatccaggtcactgaccagtcctgcagcccgcaggctctgctgtgcctctttggcgtattcctcttgctcactccccacagggatgaccaccacctggaacggggacagccacagtggccatttccccccgcagctttctgccagcactcccaacagtctttccacagaaccgagcactgctcggtgaatgaggactggacgctccagggcacccgcctgccccttatactggaggtcaaatctcaggggcagttggaagtcaagctgaattgtcccacactgatgtggccggcccagggcatcgtggaggtgcacgtcaatcttaggtccatagaaggcaccatctccagagttgaggtcccagggttctccaaattccttcagggcctgtttaaggacctgttcggcctggtcccaaaggcaagggtcccccaggaagccagatggccgggtggacagtgccaggcggaaggagaagccaagaacggcatagacggaacggaggaaatcaagacagctttggatctctgcttccagctgatctgttgtacagaagatgtgagcgtcatcctgctggaagcaccgcagtcgggtcagtccccccagaccaccagaggcttcggcccggtgtagagccccaaagtcagctagtcgcaggggcagttcccgccaggatctgggccggtgggcgaacatcaggcagtgtgcagggcagttcataggcttgagggcgagtgtatctgtgatatgcctggtagaatcgtcactctgggagctgggaggcctgtcagagcctgggggctgcacggcaaacatgtcttcctgataatgctcccagtgccctgactgttcccagagcttcgtagaaaacagtgtgggagttttcacctcggagaaaccacgatgggcatactcagccttgaacaactggcgaagctgatcccgtgaagcctctagcctccggaagggtcgagcagcagctgtaagttcctggcaaatccgctccaaaacaggcagctctgagccccggattgtcctctcctttcccaggaagaaatcatggtaaaagccatattctgtacttggacctctgcagagaacagcacctaggaattgttcagctgctgcccccaggacatgggtgctggagtgccagaacactgctttcccctctggggaatcgaatgtcagaaatctgaggtcagaatctgtctccaagggccgctccagatcataaggttctccattcacttgagcagccactgcagtatctgccagtgttgaactgatctgccgggctagttggtagggggttgtgttccatgccacagcatcaattttctggcctccaggaagtgatatcttaatagtccggggttccttctgtgccatgcttgctaatctctttacctgagcagcccacagctcctcaaaaaggccaagccgctctgccaaccagcgtggaggggtcgacacaactgccgtgtgtagcctgcaagcctgtaaaccttggagccggagacaccgccacctctgatacagggccatgttccttcacaccagtgcctacatcctcaaac

SEQ ID NO: 15405 - RNA, 2206 nt, Homo sapiens
  source 1..2206: mol_type = other RNA
gctgggattacaggcatgagccactgcgcctggcccaatttatttttttttgtagtttcattctcctcacatccaaacagctacagcttccctccttttgtggggtccccaaaccaagtctcttttcaggagagcagacatgtgcctccacacagttctgaagttctgggggctccacattgtcagctgggttggggtctcccatgtgagggaggctgatggcactcgcaggtttttgcctcatctatgtacaaaggctcagaaaatttcttcggcatttgggaccctcgtgttctgtagctccaccagtcgctgcacagcctcaggcaagtcccactccccaaggcgacgattatctcgagtccgaatgttcactgttctcttactttgctctttctggccaaccacaaactgaaaattgtagtgggcaagctgggcccggcggattctccggctgagggtcagtccagagtctgcatccaggtcactgaccagtcctgcagcccgcaggctctgctgtgcctctttggcgtattcctcttgctcactccccacagggatgaccaccacctggaacggggacagccacagtggccccttatactggaggtcaaatctcaggggcagttggaagtcaagctgaattgtcccacactgatgtggccggcccagggcatcgtggaggtgcacgtcaatcttaggtccatagaaggcaccatctccagagttgaggtcccagggttctccaaattccttcagggcctgtttaaggacctgttcggcctggtcccaaaggcaagggtcccccaggaagccagatggccgggtggacagtgccaggcggaaggagaagccaagaacggcatagacggaacggaggaaatcaagacagctttggatctctgcttccagctgatctgttgtacagaagatgtgagcgtcatcctgctggaagcaccgcagtcgggtcagtccccccagaccaccagaggcttcggcccggtgtagagccccaaagtcagctagtcgcaggggcagttcccgccaggatctgggccggtgggcgaacatcaggcagtgtgcagggcagttcataggcttgagggcgagtgtatctgtgatatgcctggtagaatcgtcactctgggagctgggaggcctgtcagagcctgggggctgcacggcaaacatgtcttcctgataatgctcccagtgccctgactgttcccagagcttcgtagaaaacagtgtgggagttttcacctcggagaaaccacgatgggcatactcagccctgataaacgccactagtgcattatacacccttgtccctcgtggcaggaagaagcagctcccagggctcagttcatggaagaagaagagctcctgttccgatagcagcttcagtcctccaatctgtccagtatgccgaaggtgggggccctggcaaaggtcaaccaatgtgccacacccatatactgttgctgttggacctgtcactttctcctcaatcaagtgaagcttaaaggggttatccttgaacaactggcgaagctgatcccgtgaagcctctagcctccggaagggtcgagcagcagctgtaagttcctggcaaatccgctccaaaacaggcagctctgagccccggattgtcctctcctttcccaggaagaaatcatggtaaaagccatattctgtacttggacctctgcagagaacagcacctaggaattgttcagctgctgcccccaggacatgggtgctggagtgccagaacactgctttcccctctggggaatcgaatgtcagaaatctgaggtcagaatctgtctccaagggccgctccagatcataaggttctccattcacttgagcagccactgcagtatctgccagtgttgaactgatctgccgggctagttggtagggggttgtgttccatgccacagcatcaattttctggcctccaggaagtgatatcttaatagtccggggttccttctgtgccatgcttgctaatctctttacctgagcagcccacagctcctcaaaaaggccaagccgctctgccaaccagcgtggaggggtcgacacaactgccgtgtgtagcctgcaagcctgtaaaccttggagccggagacaccgccacctctgatacagggccatgttccttcacaccagtgcctacatcctcaaacagattatc

SEQ ID NO: 15406 - RNA, 2353 nt, Homo sapiens
  source 1..2353: mol_type = other RNA
gctgggattacaggcatgagccactgcgcctggcccaatttatttttttttgtagtttcattctcctcacatccaaacagctacagcttccctccttttgtggggtccccaaaccaagtctcttttcaggagagcagacatgtgcctccacacagttctgaagttctgggggctccacattgtcagctgggttggggtctcccatgtgagggaggctgatggcactcgcaggtttttgcctcatctatgtacaaaggctcagaaaatttcttcggcatttgggaccctcgtgttctgtagctccaccagtcgctgcacagcctcaggcaagtcccactccccaaggcgacgattatctcgagtccgaatgttcactgttctcttactttgctctttctggccaaccacaaactgaaaattgtagtgggcaagctgggcccggcggattctccggctgagggtcagtccagagtctgcatccaggtcactgaccagtcctgcagcccgcaggctctgctgtgcctctttggcgtattcctcttgctcactccccacagggatgaccaccacctggaacggggacagccacagtggccccttatactggaggtcaaatctcaggggcagttggaagtcaagctgaattgtcccacactgatgtggccggcccagggcatcgtggaggtgcacgtcaatcttaggtccatagaaggcaccatctccagagttgaggtcccagggttctccaaattccttcagggcctgtttaaggacctgttcggcctggtcccaaaggcaagggtcccccaggaagccagatggccgggtggacagtgccaggcggaaggagaagccaagaacggcatagacggaacggaggaaatcaagacagctttggatctctgcttccagctgatctgttgtacagaagatgtgagcgtcatcctgctggaagcaccgcagtcgggtcagtccccccagaccaccagaggcttcggcccggtgtagagccccaaagtcagctagtcgcaggggcagttcccgccaggatctgggccggtgggcgaacatcaggcagtgtgcagggcagttcataggcttgagggcgagtgtatctgtgatatgcctggtagaatcgtcactctgggagctgggaggcctgtcagagcctgggggctgcacggcaaacatgtcttcctgataatgctcccagtgccctgactgttcccagagcttcgtagaaaacagtgtgggagttttcacctcggagaaaccacgatgggcatactcagccctgataaacgccactagtgcattatacacccttgtccctcgtggcaggaagaagcagctcccagggctcagttcatggaagaagaagagctcctgttccttcccaatgcgccggtggtcccgcaattctgcttcctccctccatgcttcccagaccctcagcaattctgttgtggggaaggaaatccctgacactctctgcagtgtctctggggcccctgaagacctccataaggatgatgagttcgatagcagcttcagtcctccaatctgtccagtatgccgaaggtgggggccctggcaaaggtcaaccaatgtgccacacccatatactgttgctgttggacctgtcactttctcctcaatcaagtgaagcttaaaggggttatccttgaacaactggcgaagctgatcccgtgaagcctctagcctccggaagggtcgagcagcagctgtaagttcctggcaaatccgctccaaaacaggcagctctgagccccggattgtcctctcctttcccaggaagaaatcatggtaaaagccatattctgtacttggacctctgcagagaacagcacctaggaattgttcagctgctgcccccaggacatgggtgctggagtgccagaacactgctttcccctctggggaatcgaatgtcagaaatctgaggtcagaatctgtctccaagggccgctccagatcataaggttctccattcacttgagcagccactgcagtatctgccagtgttgaactgatctgccgggctagttggtagggggttgtgttccatgccacagcatcaattttctggcctccaggaagtgatatcttaatagtccggggttccttctgtgccatgcttgctaatctctttacctgagcagcccacagctcctcaaaaaggccaagccgctctgccaaccagcgtggaggggtcgacacaactgccgtgtgtagcctgcaagcctgtaaaccttggagccggagacaccgccacctctgatacagggccatgttccttcacaccagtgcctacatcctcaaacagattatc

SEQ ID NO: 15407 - RNA, 2107 nt, Homo sapiens
  source 1..2107: mol_type = other RNA
gctgggattacaggcatgagccactgcgcctggcccaatttatttttttttgtagtttcattctcctcacatccaaacagctacagcttccctccttttgtggggtccccaaaccaagtctcttttcaggagagcagacatgtgcctccacacagttctgaagttctgggggctccacattgtcagctgggttggggtctcccatgtgagggaggctgatggcactcgcaggtttttgcctcatctatgtacaaaggctcagaaaatttcttcggcatttgggaccctcgtgttctgtagctccaccagtcgctgcacagcctcaggcaagtcccactccccaaggcgacgattatctcgagtccgaatgttcactgttctcttactttgctctttctggccaaccacaaactgaaaattgtagtgggcaagctgggcccggcggattctccggctgagggtcagtccagagtctgcatccaggtcactgaccagtcctgcagcccgcaggctctgctgtgcctctttggcgtattcctcttgctcactccccacagggatgaccaccacctggaacggggacagccacagtggccccttatactggaggtcaaatctcaggggcagttggaagtcaagctgaattgtcccacactgatgtggccggcccagggcatcgtggaggtgcacgtcaatcttaggtccatagaaggcaccatctccagagttgaggtcccagggttctccaaattccttcagggcctgtttaaggacctgttcggcctggtcccaaaggcaagggtcccccaggaagccagatggccgggtggacagtgccaggcggaaggagaagccaagaacggcatagacggaacggaggaaatcaagacagctttggatctctgcttccagctgatctgttgtacagaagatgtgagcgtcatcctgctggaagcaccgcagtcgggtcagtccccccagaccaccagaggcttcggcccggtgtagagccccaaagtcagctagtcgcaggggcagttcccgccaggatctgggccggtgggcgaacatcaggcagtgtgcagggcagttcataggcttgagggcgagtgtatctgtgatatgcctggtagaatcgtcactctgggagctgggaggcctgtcagagcctgggggctgcacggcaaacatgtcttcctgataatgctcccagtgccctgactgttcccagagcttcgtagaaaacagtgtgggagttttcacctcggagaaaccacgatgggcatactcagccgatagcagcttcagtcctccaatctgtccagtatgccgaaggtgggggccctggcaaaggtcaaccaatgtgccacacccatatactgttgctgttggacctgtcactttctcctcaatcaagtgaagcttaaaggggttatccttgaacaactggcgaagctgatcccgtgaagcctctagcctccggaagggtcgagcagcagctgtaagttcctggcaaatccgctccaaaacaggcagctctgagccccggattgtcctctcctttcccaggaagaaatcatggtaaaagccatattctgtacttggacctctgcagagaacagcacctaggaattgttcagctgctgcccccaggacatgggtgctggagtgccagaacactgctttcccctctggggaatcgaatgtcagaaatctgaggtcagaatctgtctccaagggccgctccagatcataaggttctccattcacttgagcagccactgcagtatctgccagtgttgaactgatctgccgggctagttggtagggggttgtgttccatgccacagcatcaattttctggcctccaggaagtgatatcttaatagtccggggttccttctgtgccatgcttgctaatctctttacctgagcagcccacagctcctcaaaaaggccaagccgctctgccaaccagcgtggaggggtcgacacaactgccgtgtgtagcctgcaagcctgtaaaccttggagccggagacaccgccacctctgatacagggccatgttccttcacaccagtgcctacatcctcaaacagattatc

SEQ ID NO: 15408 - RNA, 1236 nt, Homo sapiens
  source 1..1236: mol_type = other RNA
gctgggattacaggcatgagccactgcgcctggcccatttttcgatttttaacatgaggattaagtagactactacgcacatttgctaaaggcagccccttacatttctttttaagcagaaaatacttggtggttagagacagcagcgtcacagcataaccacctctaggctgtcagtgtgccctctaaaacaacagctgcacctcctctaatgtcaacccttccgtctggacgaagggaaattcccagctctcctcctcggtgggaacactgaaaagcatgcatttctttcttccccagatgctgggaccagtagctgctgagaacagcgtgtgcagaccctgtcactgggtcttcagccacaccaacccacggtgcaaaatatcttgagtaaaagtcaaatgcttgggtctgcccaccaggctctcctttaagggtaagaataagccctttcaccttccctgtgttttcaacttgcagcagattctccgtgttcactttcaggttctccagaaacgacctgttgtaaacgtcactgaggcggacgaggagcttttgggtatctggagaataacagatgtcctggaccagtgtgttgcctatggcagtctttatcaagtcctctacttcatggaagtcctgggggtgggctggataaagaggcaagtccaggacgatgccatcctctgctcgtctggcccttagttctccactcagagtgacaaacgtgagcgtgctattcatgttttttattttgtgaaacagcacagctgcagaagccagggtggcatggccacagagtgggacctcactcgctggtgtaaaccatctcagtccaaagcaggaactttgtgcaaagttgtctgtcgggtgcagttttcggataaaagcagtttcagagaggttcatctcccttgcaattttctgatgcatgtcttcatccaattcattttctaggaggcaaacagcagcaggattcccacgaaatgctcttgctgtgaatgcatctgctatgaaaataggaagcttcattttccttgcaagctgtttttgcaagttctcaaaattgctggtagcctgctttacgtcttctgggctgacgggactgcgagtgacttctgacgcagattcccaagatgagagaggctggagctgggggaggaaagccaatggcgacgaaggtgctcaactcccaaatccaggacaaaggaggcagacggcctcctttgtaattct

SEQ ID NO: 15409 - RNA, 1262 nt, Homo sapiens
  source 1..1262: mol_type = other RNA
gctgggattacaggcatgagccactgcgcctggcccatttttcgatttttaacatgaggattaagtagactactacgcacatttgctaaaggcagccccttacatttctttttaagcagaaaatacttggtggttagagacagcagcgtcacagcataaccacctctaggctgtcagtgtgccctctaaaacaacagctgcacctcctctaatgtcaacccttccgtctggacgaagggaaattcccagctctcctcctcggtgggaacactgaaaagcatgcatttctttcttccccagatgctgggaccagtagctgctgagaacagcgtgtgcagaccctgtcactgggtcttcagccacaccaacccacggtgcaaaatatcttgagtaaaagtcaaatgcttgggtctgcccaccaggctctcctttaagggtaagaataagccctttcaccttccctgtgttttcaacttgcagcagattctccgtgttcactttcaggttctccagaaacgacctgttgtaaacgtcactgaggcggacgaggagcttttgggtatctggagaataacagatgtcctggaccagtgtgttgcctatggcagtctttatcaagtcctctacttcatggaagtcctgggggtgggctggataaagaggcaagtccaggacgatgccatcctctgctcgtctggcccttagttctccactcagagtgacaaacgtgagcgtgctattcatgttttttattttgtgaaacagcacagctgcagaagccagggtggcatggccacagagtgggacctcactcgctggtgtaaaccatctcagtccaaagcaggaactttgtgcaaagttgtctgtcgggtgcagttttcggataaaagcagtttcagagaggttcatctcccttgcaattttctgatgcatgtcttcatccaattcattttctaggaggcaaacagcagcaggattcccacgaaatgctcttgctgtgaatgcatctgctatgaaaataggaagcttcattttccttgcaagctgtttttgcaagttctcaaaattgctggtagcctgctttacgtcttcttctgggctgacgggactgcgagtgacttctgacgcagattcccaagatgagagaggctggagctgggggaggaaagccaatggcgacgaaggtgctcaactcccaaatccaggacaaaggaggcagacggcctcctttgtaattctgccgcccggtggcgaagggtttt

SEQ ID NO: 15410 - RNA, 1203 nt, Homo sapiens
  source 1..1203: mol_type = other RNA
gctgggattacaggcatgagccactgcgcctggcccatttttcgatttttaacatgaggattaagtagactactacgcacatttgctaaaggcagccccttacatttctttttaagcagaaaatacttggtggttagagacagcagcgtcacagcataaccacctctaggctgtcagtgtgccctctaaaacaacagctgcacctcctctaatgtcaacccttccgtctggacgaagggaaattcccagctctcctcctcggtgggaacactgaaaagcatgcatttctttcttccccagatgctgggaccagtagctgtcactgggtcttcagccacaccaacccacggtgcaaaatatcttgagtaaaagtcaaatgcttgggtctgcccaccaggctctcctttaagggtaagaataagccctttcaccttccctgtgttttcaacttgcagcagattctccgtgttcactttcaggttctccagaaacgacctgttgtaaacgtcactgaggcggacgaggagcttttgggtatctggagaataacagatgtcctggaccagtgtgttgcctatggcagtctttatcaagtcctctacttcatggaagtcctgggggtgggctggataaagaggcaagtccaggacgatgccatcctctgctcgtctggcccttagttctccactcagagtgacaaacgtgagcgtgctattcatgttttttattttgtgaaacagcacagctgcagaagccagggtggcatggccacagagtgggacctcactcgctggtgtaaaccatctcagtccaaagcaggaactttgtgcaaagttgtctgtcgggtgcagttttcggataaaagcagtttcagagaggttcatctcccttgcaattttctgatgcatgtcttcatccaattcattttctaggaggcaaacagcagcaggattcccacgaaatgctcttgctgtgaatgcatctgctatgaaaataggaagcttcattttccttgcaagctgtttttgcaagttctcaaaattgctggtagcctgctttacgtcttctgggctgacgggactgcgagtgacttctgacgcagattcccaagatgagagaggctggagctgggggaggaaagccaatggcgacgaaggtgctcaactcccaaatccaggacaaaggaggcagacggcctccttt

SEQ ID NO: 15411 - RNA, 1237 nt, Homo sapiens
  source 1..1237: mol_type = other RNA
gctgggattacaggcatgagccactgcgcctggcccatttttcgatttttaacatgaggattaagtagactactacgcacatttgctaaaggcagccccttacatttctttttaagcagaaaatacttggtggttagagacagcagcgtcacagcataaccacctctaggctgtcagtgtgccctctaaaacaacagctgcacctcctctaatgtcaacccttccgtctggacgaagggaaattcccagctctcctcctcggtgggaacactgaaaagcatgcatttctttcttccccagatgctgggaccagtagctgtcactgggtcttcagccacaccaacccacggtgcaaaatatcttgagtaaaagtcaaatgcttgggtctgcccaccaggctctcctttaagggtaagaataagccctttcaccttccctgtgttttcaacttgcagcagattctccgtgttcactttcaggttctccagaaacgacctgttgtaaacgtcactgaggcggacgaggagcttttgggtatctggagaataacagatgtcctggaccagtgtgttgcctatggcagtctttatcaagtcctctacttcatggaagtcctgggggtgggctggataaagaggcaagtccaggacgatgccatcctctgctcgtctggcccttagttctccactcagagtgacaaacgtgagcgtgctattcatgttttttattttgtgaaacagcacagctgcagaagccagggtggcatggccacagagtgggacctcactcgctggtgtaaaccatctcagtccaaagcaggaactttgtgcaaagttgtctgtcgggtgcagttttcggataaaagcagtttcagagaggttcatctcccttgcaattttctgatgcatgtcttcatccaattcattttctaggaggcaaacagcagcaggattcccacgaaatgctcttgctgtgaatgcatctgctatgaaaataggaagcttcattttccttgcaagctgtttttgcaagttctcaaaattgctggtagcctgctttacgtcttcttctgggctgacgggactgcgagtgacttctgacgcagattcccaagatgagagaggctggagctgggggaggaaagccaatggcgacgaaggtgctcaactcccaaatccaggacaaaggaggcagacggcctcctttgtaattctgccgcccggtggcgaagggtttt

SEQ ID NO: 15412 - RNA, 2524 nt, Homo sapiens
  source 1..2524: mol_type = other RNA
gctgggattacaggcatgagccactgcgcctggccccaactggcttattttctgtcaaactcagtgtttgatagaaacagtctagtatgtcaggttctctttttaaccttactgattccagaggccacaatggaggggaaaaggctagcataaggaagagtttcctcaaatgccttctctaggctacgatttttatgtaaaggctgattaagtggtttgctgggatctggagctgcccaaggaatttctgcccactcggaaggccactggtgtcctgagtgttgctcattcagcagaatgaagcgctctgtcaagctgtgaaggccactggtgggggaaagagggaatatgctcattcttgttattgctgttgctattaataaacagggctttatggattaaaaggggagagagctatgacattattaacattaattcttcttcattaactaatctttgaattttttaggtttttttttctctttaggacacataagcccagccaagattcaaaggcttccttttataaactaaagtacaatatttctgtgtcattattatatatagccttgagtaatcacaattaatgtgatttttaatgcacaaattaaacatgctataaactctaatgatgatcatgcaggattttgatcactatcatcattaggtgaaacctcagaaaaaaatgtaagcctatcatgggtcctaacagctttttattttaattctacagatttgggcatattggctgttgagagagagaaaaccaaaaccttctctttttccatctggctatgagtgcttttcatagcttattttttccacactcacccctaaaaaatgcactggagctgagctattgtaagaatgtgtcagattcaaatgattatatcattgactatctgctatttcacaggagaactgaactgtctgactttttaaaaaactcagcacggactttatagtagcgagactttatcaacagtgagttagtgttacaggtgacttggctcataaaaaattaaaagcttcagaaattaactttatcacagaaaacatttagtcataagcaacccccagttgtagaggcagagaaccaaagatcagagatatgtgccaaaaaatacttttcagaccccgagcaaagagaatagtaagagctggtgtcagcccattgcggtgccaggctgagctagctggtaaggtctctggtaaagaaaacgcttttctgggacgactataatgggcactctgtgagctccggggcctggagttgcttttcgacagatgactttgttccttctttacatggtaaagttcagtttatatttttgtagaaatacattcttgacatttccaatgaaaatgctgacttggtcgcattttagtttcattctaattggaagaaatgagccctcgcttgtttggaaaacaaaaggctacgaaaactcgtgttcattttgggaacttttattaagtattcaaaacagaatgaaagtgatctagttctggaaaagcagggtcatatctaaaattaaaaacaaaaactaggttgctgagagagatcaaaagacaaaaggaattcactaagcagatgaaagttaaaaacacggcatatataacctcatcacctgaggtacgctgatttaatatcagcagcgccaacaaaaaaagtaaaatcataatgggctcccatctctccaaaagcaaatcaatgcctcattgtgaaaagaaacccacaaagagatggtgattttacttttatttcaaagaccaaataaagtctttggtcctgtaagcaagttttaatactgtaacaagattgctaacttttgctgtcagtctgactcataaaggacttaattacttttttcgacagtcaagaagggtccactcagagaaattgtgtggcagagaaaaaagggcagcgtggccaagaggaacctgtaatgatgcactcgtcaattacagctatttctttcaaacttgtcttgttaaatttaccttcctttccagacgtcataaattagccctccattaaagcatctgaatgccaaacagtacattattcttcacaaggtgaccatcaggagcaggctatgctggaattgtattcttttccaattggctgctaatatcaccactcctggttcttcctttctttcttgattcaagagcctcttcccatcacctgaattgcttcaataaagacacagacttaatttgtggttcttcaataaattcaaagagaaagttacaacgtgcattgaagagacacattcttgttaaaaggcattgtgggaagccaccattcttggtggtggattccagcaccttgaaacaccacaaactggaagagcaagcaaggagccaatggctaattctaccacagacaactatgctcagcaagggtgagctaagggaattaaggatacaataaaataatggggccaagcatggtggctcacgcctgtaatcccagcactttgggaggccgaggtgggtggatcatgaggtcaagagc

SEQ ID NO: 15413 - RNA, 2643 nt, Homo sapiens
  source 1..2643: mol_type = other RNA
gctgggattacaggcatgagccactgcgcctggccgagtagagaagaatttactgctgattaaggttgtgtttttcaacctgcaatcccgagaccctcagaataaagattacttgaggttgctatgaaaaatacagattcctgtcctccccctggctgaatcagaatctcataaggtgaggctcaggtttctgcacttttcacaagctctgtaatggttacagtgcaccctaatgtttgagaaccagtggcctaaagagaatgcaacctaagagggcaaggctagtgcatagcttaaatcgctccagcctttggtaatcccttctaaacacagtaccacccatgtggaggagactgcaaggaagctgttattcaaagtagaacagtcagccttgtgcttgagtcctgctttatgcttgcgtgtttcataacaaaacacaaaggcaagtcttcatatcagcacttagtcttgatatccaagtagctgactactgtacttatgataacagcttgaagaggactgcaactctcccctcacgaatggtgacagagttggcttgtcacacctggctcagggaagaaaaatgagtaaacccctacctctttactcttgattcctcttccaccctaatactgttaacacatcatcctgtgtgattcaaataatctggcagatgaaatacagaaaatctaagtcatattgttcttatcactctatggccagatattatactaatctaattttaaaaatccttttctgtgcaatagaaataaccaaagctcattctgtctcctttcctttctaatgctgttgataggaacaaaatatcaagtaaggatacatgctagagatgttaaattcatacaagtaaagtaaattacaaagagaggtggtaatatttttttctagaatttcacaataaaatccctctcaccatgaaaatctttttataattttaacaggaaacttaaaagacattttgttgcaagactatcttaacaattataagaataatgccattatctgtgctcaatatagataaacataacagtaactttaaaaggccaagtatactcataagtgaggatgaaatttatttttcaacaaccaatatgccaatatccaacttctaggttttattcaattctaatgtcatgggtttctcctaccccagtcaaaactcctgccaaatgtccacaaaattgacaccaaaatcaacaaacacaaagaaagagagggacagggagagggaaagagaaatagagagtgaggaaggaaggaacgtgacaagagctaccatgcaaaatgaccagaagaactggagttcagtggcacagatcagcaggagcagaggaatgctgcaaaagatgatgctgcatagagtctaacttggagatgcctgtatgatgctggatgaccaagtactaaggtcacaagtgtgttcatggacccataagaaccaggatcttgacccaaacttataagatcttctaaaaagaaaatacttcatctaaattgaagcaattcctaagtcaaacaccagaagagttccttatttgatgtaagttgtgcctaaaactttggctgatacaaagaaacccgtccactaaggcaccctgaggcaatctgacaatgtgttggagagaactttgttgtcagtaccacatcattatgagagtacagagaacggatcacccgcaggggactggcttctttgggcaagcagtcaacaagttcactgcactgtttgtcaaatcccaacaagcgaatcccatagccatgtggggaagaaatcattcgtccatcggggctgaagcaaagttctttgatgtaacccctgcctacattggcttcttcaatgtaatgagtcagtcgtagagaacagcgaggtgagacaggtcgcactggagctccttcttggaattcatagacacaagtacactcctcatcatcactgttgcttgagcaccgaagaagagtggcccagccttttgggtgcagctgtaaggacgtgatgcagtttccgtggtcactctcaccaagaacttcaggggttacgacttcaagactatttcgtggtgaaactccttctctttgagaggctcgtgacatgtgtttctcagaagaattagaatcactatgatgacaaggtgagccagaaactctaggaccagatgaacttgatgaagtggtcaaatctgaacttgaagtagttcttcttgctcttaaaatgggatagctgcctacttctaaagacttagttaagtcaaggtcatgcaaaattaagagatatccagaggacgttgaaatcaacattttggaacaatctggtgttaacctcattcgcatgagaaaacgtgtgtgaaagaatttcttatgtggacacccatcttctgtatacctgatattatttacacagtcttcatgagcttcagaaagtgtttttatgtgctttgaagatatagggtcaaaaagcagaacttcagtttgttcacaagcaactgtcagcactgactgtgtaccagaaagccctagttgtgggctggctctgacaggtccgctgtgtagcttcgggcatttctccttcacagagcccaagtcctgaaggcgagcaagtggggccccgcctgcctgcctcaaaaa

SEQ ID NO: 15414 - RNA, 3322 nt, Homo sapiens
  source 1..3322: mol_type = other RNA
gctgggattacaggcatgagccactgcgcctggccgagtagagaagaatttactgctgattaaggttgtgtttttcaacctgcaatcccgagaccctcagaataaagattacttgaggttgctatgaaaaatacagattcctgtcctccccctggctgaatcagaatctcataaggtgaggctcaggtttctgcacttttcacaagctctgtaatggttacagtgcaccctaatgtttgagaaccagtggcctaaagagaatgcaacctaagagggcaaggctagtgcatagcttaaatcgctccagcctttggtaatcccttctaaacacagtaccacccatgtggaggagactgcaaggaagctgttattcaaagtagaacagtcagccttgtgcttgagtcctgctttatgcttgcgtgtttcataacaaaacacaaaggcaagtcttcatatcagcacttagtcttgatatccaagtagctgactactgtacttatgataacagcttgaagaggactgcaactctcccctcacgaatggtgacagagttggcttgtcacacctggctcagggaagaaaaatgagtaaacccctacctctttactcttgattcctcttccaccctaatactgttaacacatcatcctgtgtgattcaaataatctggcagatgaaatacagaaaatctaagtcatattgttcttatcactctatggccagatattatactaatctaattttaaaaatccttttctgtgcaatagaaataaccaaagctcattctgtctcctttcctttctaatgctgttgataggaacaaaatatcaagtaaggatacatgctagagatgttaaattcatacaagtaaagtaaattacaaagagaggtggtaatatttttttctagaatttcacaataaaatccctctcaccatgaaaatctttttataattttaacaggaaacttaaaagacattttgttgcaagactatcttaacaattataagaataatgccattatctgtgctcaatatagataaacataacagtaactttaaaaggccaagtatactcataagtgaggatgaaatttatttttcaacaaccaatatgccaatatccaacttctaggttttattcaattctaatgtcatgggtttctcctaccccagtcaaaactcctgccaaatgtccacaaaattgacaccaaaatcaacaaacacaaagaaagagagggacagggagagggaaagagaaatagagagtgaggaaggaaggaacgtgacaagagctaccatgcaaaatgaccagaagaactggagttcagtggcacagatcagcaggagcagaggaatgctgcaaaagatgatgctgcatagagtctaacttggagatgcctgtatgatgctggatgaccaagtactaaggtcacaagtgtgttcatggacccataagaaccaggatcttgacccaaacttataagatcttctaaaaagaaaatacttcatctaaattgaagcaattcctaagtcaaacaccagaagagttccttatttgatgtaagttgtgcctaaaactttggctgatacaaagaaacccgtccactaaggcaccctgaggcaatctgacaatgtgttggagagaactttgttgtcagtaccacatcattatgagagtacagagaacggatcacccgcaggggactggcttctttgggcaagcagtcaacaagttcactgcactgtttgtcaaatcccaacaagcgaatcccatagccatgtggggaagaaatcattcgtccatcggggctgaagcaaagttctttgatgtaacccctgcctacattggcttcttcaatgtaatgagtcagtcgtagagaacagcgaggtgagacaggtcgcactggagctccttcttggaattcatagacacaagtacactcctcatcatcactgttgcttgagcaccgaagaagagtggcccagccttttgggtgcagctgtaaggacgtgatgcagtttccgtggtcactctcaccaagaacttcaggggttacgacttcaagactatttcgtggtgaaactccttctctttgagaggctcgtgacatgtgtttctcagaagaattagaatcactatgatgacaaggtgagccagaaactctaggaccagatgaacttgatgaagtggtcaaatctgaacttgaagtagttcttcttgctcttaaaatgggatagctgcctacttctaaagacttagttaagtcaaggtcatgcaaaattaagagatatccagaggacgttgaaatcaacattttggaacaatctggtgttaacctcattcgcatgagaaaacgtgtgtgaaagaatttcttatgtggacacccatcttctgtatacctgttagtgtcccaaataatgacatttccatcaaatcctgatgttactaagagtcttgtattagtatcatattcgatgttcttcacccagctagtgtgaccatgtaaagtgcatactttggtgttcaattttctcagatcccatagtgctattgtagtgtcatcagagcaggtagcaaacagccggttatcaagaaatctgatattatttacacagtcttcatgagcttcagaaagtgtttttatgtgctttgaagatatagggtcaaaaagcagaacttcagtttgttcacaagcaactgtcagcactgacccgtcgggcgagtactcgaggttgaagacggcgccgtgggtgcgggtgctgaggtacaccgagtccgcggggtggatggaaccgtagaggctagtcatggtgcgaaaattgtcccgcgccgggtccacgaacagcccgcggcccaggctgcgctctttcagccacccgaacagcctagcgccagggccgcccaggcccgcgccgaggccgtgtcggccccggctcttggccctgcagtctggcccgggccgccggcacggaggggagggaggtgacggctctcccggggcggaggcagttgaggactccggagctccaggcagccctagctctccggagcgcggggccggggacagcgatggggcgccggggcggcgagggcttcgggcgggtggagggggatgggtcgcatcagccccgggatgtagtggcgagggcggcccggtggctgctgcctgcccctcgtggggcgtcggctcctcagccccggctccggccgatccgtcccctccagggctatggggcccaaagggaaacatgatcaacgcccccgccccccgctccgggccactgccccgccggccgacacctcagtgcccctgttcagct

SEQ ID NO: 15415 - RNA, 2807 nt, Homo sapiens
  source 1..2807: mol_type = other RNA
gctgggattacaggcatgagccactgcgcctggccgagtagagaagaatttactgctgattaaggttgtgtttttcaacctgcaatcccgagaccctcagaataaagattacttgaggttgctatgaaaaatacagattcctgtcctccccctggctgaatcagaatctcataaggtgaggctcaggtttctgcacttttcacaagctctgtaatggttacagtgcaccctaatgtttgagaaccagtggcctaaagagaatgcaacctaagagggcaaggctagtgcatagcttaaatcgctccagcctttggtaatcccttctaaacacagtaccacccatgtggaggagactgcaaggaagctgttattcaaagtagaacagtcagccttgtgcttgagtcctgctttatgcttgcgtgtttcataacaaaacacaaaggcaagtcttcatatcagcacttagtcttgatatccaagtagctgactactgtacttatgataacagcttgaagaggactgcaactctcccctcacgaatggtgacagagttggcttgtcacacctggctcagggaagaaaaatgagtaaacccctacctctttactcttgattcctcttccaccctaatactgttaacacatcatcctgtgtgattcaaataatctggcagatgaaatacagaaaatctaagtcatattgttcttatcactctatggccagatattatactaatctaattttaaaaatccttttctgtgcaatagaaataaccaaagctcattctgtctcctttcctttctaatgctgttgataggaacaaaatatcaagtaaggatacatgctagagatgttaaattcatacaagtaaagtaaattacaaagagaggtggtaatatttttttctagaatttcacaataaaatccctctcaccatgaaaatctttttataattttaacaggaaacttaaaagacattttgttgcaagactatcttaacaattataagaataatgccattatctgtgctcaatatagataaacataacagtaactttaaaaggccaagtatactcataagtgaggatgaaatttatttttcaacaaccaatatgccaatatccaacttctaggttttattcaattctaatgtcatgggtttctcctaccccagtcaaaactcctgccaaatgtccacaaaattgacaccaaaatcaacaaacacaaagaaagagagggacagggagagggaaagagaaatagagagtgaggaaggaaggaacgtgacaagagctaccatgcaaaatgaccagaagaactggagttcagtggcacagatcagcaggagcagaggaatgctgcaaaagatgatgctgcatagagtctaacttggagatgcctgtatgatgctggatgaccaagtactaaggtcacaagtgtgttcatggacccataagaaccaggatcttgacccaaacttataagatcttctaaaaagaaaatacttcatctaaattgaagcaattcctaagtcaaacaccagaagagttccttatttgatgtaagttgtgcctaaaactttggctgatacaaagaaacccgtccactaaggcaccctgaggcaatctgacaatgtgttggagagaactttgttgtcagtaccacatcattatgagagtacagagaacggatcacccgcaggggactggcttctttgggcaagcagtcaacaagttcactgcactgtttgtcaaatcccaacaagcgaatcccatagccatgtggggaagaaatcattcgtccatcggggctgaagcaaagttctttgatgtaacccctgcctacattggcttcttcaatgtaatgagtcagtcgtagagaacagcgaggtgagacaggtcgcactggagctccttcttggaattcatagacacaagtacactcctcatcatcactgttgcttgagcaccgaagaagagtggcccagccttttgggtgcagctgtaaggacgtgatgcagtttccgtggtcactctcaccaagaacttcaggggttacgacttcaagactatttcgtggtgaaactccttctctttgagaggctcgtgacatgtgtttctcagaagaattagaatcactatgatgacaaggtgagccagaaactctaggaccagatgaacttgatgaagtggtcaaatctgaacttgaagtagttcttcttgctcttaaaatgggatagctgcctacttctaaagacttagttaagtcaaggtcatgcaaaattaagagatatccagaggacgttgaaatcaacattttggaacaatctggtgttaacctcattcgcatgagaaaacgtgtgtgaaagaatttcttatgtggacacccatcttctgtatacctgttagtgtcccaaataatgacatttccatcaaatcctgatgttactaagagtcttgtattagtatcatattcgatgttcttcacccagctagtgtgaccatgtaaagtgcatactttggtgttcaattttctcagatcccatagtgctattgtagtgtcatcagagcaggtagcaaacagccggttatcaagaaatctgatattatttacacagtcttcatgagcttcagaaagtgtttttatgtgctttgaagatatagggtcaaaaagcagaacttcagtttgttcacaagcaactgtcagcactgacctgtgtgagcgactgagcatctgggcacctgatctgggtggcagagtcggtctgtagttgtcagtgaccggtggccgcgtgcctggggatgagt

SEQ ID NO: 15416 - RNA, 3527 nt, Homo sapiens
  source 1..3527: mol_type = other RNA
gctgggattacaggcatgagccactgcgcctggccgagtagagaagaatttactgctgattaaggttgtgtttttcaacctgcaatcccgagaccctcagaataaagattacttgaggttgctatgaaaaatacagattcctgtcctccccctggctgaatcagaatctcataaggtgaggctcaggtttctgcacttttcacaagctctgtaatggttacagtgcaccctaatgtttgagaaccagtggcctaaagagaatgcaacctaagagggcaaggctagtgcatagcttaaatcgctccagcctttggtaatcccttctaaacacagtaccacccatgtggaggagactgcaaggaagctgttattcaaagtagaacagtcagccttgtgcttgagtcctgctttatgcttgcgtgtttcataacaaaacacaaaggcaagtcttcatatcagcacttagtcttgatatccaagtagctgactactgtacttatgataacagcttgaagaggactgcaactctcccctcacgaatggtgacagagttggcttgtcacacctggctcagggaagaaaaatgagtaaacccctacctctttactcttgattcctcttccaccctaatactgttaacacatcatcctgtgtgattcaaataatctggcagatgaaatacagaaaatctaagtcatattgttcttatcactctatggccagatattatactaatctaattttaaaaatccttttctgtgcaatagaaataaccaaagctcattctgtctcctttcctttctaatgctgttgataggaacaaaatatcaagtaaggatacatgctagagatgttaaattcatacaagtaaagtaaattacaaagagaggtggtaatatttttttctagaatttcacaataaaatccctctcaccatgaaaatctttttataattttaacaggaaacttaaaagacattttgttgcaagactatcttaacaattataagaataatgccattatctgtgctcaatatagataaacataacagtaactttaaaaggccaagtatactcataagtgaggatgaaatttatttttcaacaaccaatatgccaatatccaacttctaggttttattcaattctaatgtcatgggtttctcctaccccagtcaaaactcctgccaaatgtccacaaaattgacaccaaaatcaacaaacacaaagaaagagagggacagggagagggaaagagaaatagagagtgaggaaggaaggaacgtgacaagagctaccatgcaaaatgaccagaagaactggagttcagtggcacagatcagcaggagcagaggaatgctgcaaaagatgatgctgcatagagtctaacttggagatgcctgtatgatgctggatgaccaagtactaaggtcacaagtgtgttcatggacccataagaaccaggatcttgacccaaacttataagatcttctaaaaagaaaatacttcatctaaattgaagcaattcctaagtcaaacaccagaagagttccttatttgatgtaagttgtgcctaaaactttggctgatacaaagaaacccgtccactaaggcaccctgaggcaatctgacaatgtgttggagagaactttgttgtcagtaccacatcattatgagagtacagagaacggatcacccgcaggggactggcttctttgggcaagcagtcaacaagttcactgcactgtttgtcaaatcccaacaagcgaatcccatagccatgtggggaagaaatcattcgtccatcggggctgaagcaaagttctttgatgtaacccctgcctacattggcttcttcaatgtaatgagtcagtcgtagagaacagcgaggtgagacaggtcgcactggagctccttcttggaattcatagacacaagtacactcttcccctacacaattcaaaggctcttctcttctctcctttcagttgtggcctctaggaccagtgagatccttggaagactcttgctttccagagtgatgagaatcataaagtcatttaacacctttccccctagtcatcagtatagtcccttcctttcccagagtttcccctcctcatcatcactgttgcttgagcaccgaagaagagtggcccagccttttgggtgcagctgtaaggacgtgatgcagtttccgtggtcactctcaccaagaacttcaggggttacgacttcaagactatttcgtggtgaaactccttctctttgagaggctcgtgacatgtgtttctcagaagaattagaatcactatgatgacaaggtgagccagaaactctaggaccagatgaacttgatgaagtggtcaaatctgaacttgaagtagttcttcttgctcttaaaatgggatagctgcctacttctaaagacttagttaagtcaaggtcatgcaaaattaagagatatccagaggacgttgaaatcaacattttggaacaatctggtgttaacctcattcgcatgagaaaacgtgtgtgaaagaatttcttatgtggacacccatcttctgtatacctgttagtgtcccaaataatgacatttccatcaaatcctgatgttactaagagtcttgtattagtatcatattcgatgttcttcacccagctagtgtgaccatgtaaagtgcatactttggtgttcaattttctcagatcccatagtgctattgtagtgtcatcagagcaggtagcaaacagccggttatcaagaaatctgatattatttacacagtcttcatgagcttcagaaagtgtttttatgtgctttgaagatatagggtcaaaaagcagaacttcagtttgttcacaagcaactgtcagcactgacccgtcgggcgagtactcgaggttgaagacggcgccgtgggtgcgggtgctgaggtacaccgagtccgcggggtggatggaaccgtagaggctagtcatggtgcgaaaattgtcccgcgccgggtccacgaacagcccgcggcccaggctgcgctctttcagccacccgaacagcctagcgccagggccgcccaggcccgcgccgaggccgtgtcggccccggctcttggccctgcagtctggcccgggccgccggcacggaggggagggaggtgacggctctcccggggcggaggcagttgaggactccggagctccaggcagccctagctctccggagcgcggggccggggacagcgatggggcgccggggcggcgagggcttcgggcgggtggagggggatgggtcgcatcagccccgggatgtagtggcgagggcggcccggtggctgctgcctgcccctcgtggggcgtcggctcctcagccccggctccggccgatccgtcccctccagggctatggggcccaaagggaaacatgatcaacgcccccgccccccgctccgggccactgccccgccggccgacacctcagtgcccctgttcagctgccacttccggcgtgcagcggcctaaccccac

SEQ ID NO: 15417 - RNA, 3652 nt, Homo sapiens
  source 1..3652: mol_type = other RNA
gctgggattacaggcatgagccactgcgcctggccgagtagagaagaatttactgctgattaaggttgtgtttttcaacctgcaatcccgagaccctcagaataaagattacttgaggttgctatgaaaaatacagattcctgtcctccccctggctgaatcagaatctcataaggtgaggctcaggtttctgcacttttcacaagctctgtaatggttacagtgcaccctaatgtttgagaaccagtggcctaaagagaatgcaacctaagagggcaaggctagtgcatagcttaaatcgctccagcctttggtaatcccttctaaacacagtaccacccatgtggaggagactgcaaggaagctgttattcaaagtagaacagtcagccttgtgcttgagtcctgctttatgcttgcgtgtttcataacaaaacacaaaggcaagtcttcatatcagcacttagtcttgatatccaagtagctgactactgtacttatgataacagcttgaagaggactgcaactctcccctcacgaatggtgacagagttggcttgtcacacctggctcagggaagaaaaatgagtaaacccctacctctttactcttgattcctcttccaccctaatactgttaacacatcatcctgtgtgattcaaataatctggcagatgaaatacagaaaatctaagtcatattgttcttatcactctatggccagatattatactaatctaattttaaaaatccttttctgtgcaatagaaataaccaaagctcattctgtctcctttcctttctaatgctgttgataggaacaaaatatcaagtaaggatacatgctagagatgttaaattcatacaagtaaagtaaattacaaagagaggtggtaatatttttttctagaatttcacaataaaatccctctcaccatgaaaatctttttataattttaacaggaaacttaaaagacattttgttgcaagactatcttaacaattataagaataatgccattatctgtgctcaatatagataaacataacagtaactttaaaaggccaagtatactcataagtgaggatgaaatttatttttcaacaaccaatatgccaatatccaacttctaggttttattcaattctaatgtcatgggtttctcctaccccagtcaaaactcctgccaaatgtccacaaaattgacaccaaaatcaacaaacacaaagaaagagagggacagggagagggaaagagaaatagagagtgaggaaggaaggaacgtgacaagagctaccatgcaaaatgaccagaagaactggagttcagtggcacagatcagcaggagcagaggaatgctgcaaaagatgatgctgcatagagtctaacttggagatgcctgtatgatgctggatgaccaagtactaaggtcacaagtgtgttcatggacccataagaaccaggatcttgacccaaacttataagatcttctaaaaagaaaatacttcatctaaattgaagcaattcctaagtcaaacaccagaagagttccttatttgatgtaagttgtgcctaaaactttggctgatacaaagaaacccgtccactaaggcaccctgaggcaatctgacaatgtgttggagagaactttgttgtcagtaccacatcattatgagagtacagagaacggatcacccgcaggggactggcttctttgggcaagcagtcaacaagttcactgcactgtttgtcaaatcccaacaagcgaatcccatagccatgtggggaagaaatcattcgtccatcggggctgaagcaaagttctttgatgtaacccctgcctacattggcttcttcaatgtaatgagtcagtcgtagagaacagcgaggtgagacaggtcgcactggagctccttcttggaattcatagacacaagtacactcttcccctacacaattcaaaggctcttctcttctctcctttcagttgtggcctctaggaccagtgagatccttggaagactcttgctttccagagtgatgagaatcataaagtcatttaacacctttccccctagtcatcagtatagtcccttcctttcccagagtttcccctggtttttaaaaaaagaaaattatgatactcaattggcttagtaaaatctcacatttagccagcttagctgaaacatttcagacctatgtttattatacaaggggtttttgtttgtttgtttgtttgtttgtttagggtgagatgaaagaggcaagatttaagaagctgggcaaaaactgagctgatgctggcctttaaagtacctcccaccttgctcaaccccagcaggagaggaataagaagagtttggaagggataatgataccatatgaagcaagagaggacagaaacaggagagtcgagaagcaggatctctagcagtatgcccttgaaggcagagactgcagtcagcgatcggcctaagctctgcacacacggcaatggcaatttgtccaatgagccctgttgaaggtggagtgctgctgcctgtacctcctcatcatcactgttgcttgagcaccgaagaagagtggcccagccttttgggtgcagctgtaaggacgtgatgcagtttccgtggtcactctcaccaagaacttcaggggttacgacttcaagactatttcgtggtgaaactcctgaacttgaagtagttcttcttgctcttaaaatgggatagctgcctacttctaaagacttagttaagtcaaggtcatgcaaaattaagagatatccagaggacgttgaaatcaacattttggaacaatctggtgttaacctcattcgcatgagaaaacgtgtgtgaaagaatttcttatgtggacacccatcttctgtatacctgatattatttacacagtcttcatgagcttcagaaagtgtttttatgtgctttgaagatatagggtcaaaaagcagaacttcagtttgttcacaagcaactgtcagcactgacccgtcgggcgagtactcgaggttgaagacggcgccgtgggtgcgggtgctgaggtacaccgagtccgcggggtggatggaaccgtagaggctagtcatggtgcgaaaattgtcccgcgccgggtccacgaacagcccgcggcccaggctgcgctctttcagccacccgaacagcctagcgccagggccgcccaggcccgcgccgaggccgtgtcggccccggctcttggccctgcagtctggcccgggccgccggcacggaggggagggaggtgacggctctcccggggcggaggcagttgaggactccggagctccaggcagccctagctctccggagcgcggggccggggacagcgatggggcgccggggcggcgagggcttcgggcgggtggagggggatgggtcgcatcagccccgggatgtagtggcgagggcggcccggtggctgctgcctgcccctcgtggggcgtcggctcctcagccccggctccggccgatccgtcccctccagggctatggggcccaaagggaaacatgatcaacgcccccgccccccgctccgggccactgccccgccggccgacacctcagtgcccctgttcagctgccacttccggcgtgcagcggcctaaccccac

SEQ ID NO: 15418 - RNA, 3850 nt, Homo sapiens
  source 1..3850: mol_type = other RNA
gctgggattacaggcatgagccactgcgcctggccgagtagagaagaatttactgctgattaaggttgtgtttttcaacctgcaatcccgagaccctcagaataaagattacttgaggttgctatgaaaaatacagattcctgtcctccccctggctgaatcagaatctcataaggtgaggctcaggtttctgcacttttcacaagctctgtaatggttacagtgcaccctaatgtttgagaaccagtggcctaaagagaatgcaacctaagagggcaaggctagtgcatagcttaaatcgctccagcctttggtaatcccttctaaacacagtaccacccatgtggaggagactgcaaggaagctgttattcaaagtagaacagtcagccttgtgcttgagtcctgctttatgcttgcgtgtttcataacaaaacacaaaggcaagtcttcatatcagcacttagtcttgatatccaagtagctgactactgtacttatgataacagcttgaagaggactgcaactctcccctcacgaatggtgacagagttggcttgtcacacctggctcagggaagaaaaatgagtaaacccctacctctttactcttgattcctcttccaccctaatactgttaacacatcatcctgtgtgattcaaataatctggcagatgaaatacagaaaatctaagtcatattgttcttatcactctatggccagatattatactaatctaattttaaaaatccttttctgtgcaatagaaataaccaaagctcattctgtctcctttcctttctaatgctgttgataggaacaaaatatcaagtaaggatacatgctagagatgttaaattcatacaagtaaagtaaattacaaagagaggtggtaatatttttttctagaatttcacaataaaatccctctcaccatgaaaatctttttataattttaacaggaaacttaaaagacattttgttgcaagactatcttaacaattataagaataatgccattatctgtgctcaatatagataaacataacagtaactttaaaaggccaagtatactcataagtgaggatgaaatttatttttcaacaaccaatatgccaatatccaacttctaggttttattcaattctaatgtcatgggtttctcctaccccagtcaaaactcctgccaaatgtccacaaaattgacaccaaaatcaacaaacacaaagaaagagagggacagggagagggaaagagaaatagagagtgaggaaggaaggaacgtgacaagagctaccatgcaaaatgaccagaagaactggagttcagtggcacagatcagcaggagcagaggaatgctgcaaaagatgatgctgcatagagtctaacttggagatgcctgtatgatgctggatgaccaagtactaaggtcacaagtgtgttcatggacccataagaaccaggatcttgacccaaacttataagatcttctaaaaagaaaatacttcatctaaattgaagcaattcctaagtcaaacaccagaagagttccttatttgatgtaagttgtgcctaaaactttggctgatacaaagaaacccgtccactaaggcaccctgaggcaatctgacaatgtgttggagagaactttgttgtcagtaccacatcattatgagagtacagagaacggatcacccgcaggggactggcttctttgggcaagcagtcaacaagttcactgcactgtttgtcaaatcccaacaagcgaatcccatagccatgtggggaagaaatcattcgtccatcggggctgaagcaaagttctttgatgtaacccctgcctacattggcttcttcaatgtaatgagtcagtcgtagagaacagcgaggtgagacaggtcgcactggagctccttcttggaattcatagacacaagtacactcttcccctacacaattcaaaggctcttctcttctctcctttcagttgtggcctctaggaccagtgagatccttggaagactcttgctttccagagtgatgagaatcataaagtcatttaacacctttccccctagtcatcagtatagtcccttcctttcccagagtttcccctggtttttaaaaaaagaaaattatgatactcaattggcttagtaaaatctcacatttagccagcttagctgaaacatttcagacctatgtttattatacaaggggtttttgtttgtttgtttgtttgtttgtttagggtgagatgaaagaggcaagatttaagaagctgggcaaaaactgagctgatgctggcctttaaagtacctcccaccttgctcaaccccagcaggagaggaataagaagagtttggaagggataatgataccatatgaagcaagagaggacagaaacaggagagtcgagaagcaggatctctagcagtatgcccttgaaggcagagactgcagtcagcgatcggcctaagctctgcacacacggcaatggcaatttgtccaatgagccctgttgaaggtggagtgctgctgcctgtacctcctcatcatcactgttgcttgagcaccgaagaagagtggcccagccttttgggtgcagctgtaaggacgtgatgcagtttccgtggtcactctcaccaagaacttcaggggttacgacttcaagactatttcgtggtgaaactcctgaacttgaagtagttcttcttgctcttaaaatgggatagctgcctacttctaaagacttagttaagtcaaggtcatgcaaaattaagagatatccagaggacgttgaaatcaacattttggaacaatctggtgttaacctcattcgcatgagaaaacgtgtgtgaaagaatttcttatgtggacacccatcttctgtatacctgttagtgtcccaaataatgacatttccatcaaatcctgatgttactaagagtcttgtattagtatcatattcgatgttcttcacccagctagtgtgaccatgtaaagtgcatactttggtgttcaattttctcagatcccatagtgctattgtagtgtcatcagagcaggtagcaaacagccggttatcaagaaatctgatattatttacacagtcttcatgagcttcagaaagtgtttttatgtgctttgaagatatagggtcaaaaagcagaacttcagtttgttcacaagcaactgtcagcactgacccgtcgggcgagtactcgaggttgaagacggcgccgtgggtgcgggtgctgaggtacaccgagtccgcggggtggatggaaccgtagaggctagtcatggtgcgaaaattgtcccgcgccgggtccacgaacagcccgcggcccaggctgcgctctttcagccacccgaacagcctagcgccagggccgcccaggcccgcgccgaggccgtgtcggccccggctcttggccctgcagtctggcccgggccgccggcacggaggggagggaggtgacggctctcccggggcggaggcagttgaggactccggagctccaggcagccctagctctccggagcgcggggccggggacagcgatggggcgccggggcggcgagggcttcgggcgggtggagggggatgggtcgcatcagccccgggatgtagtggcgagggcggcccggtggctgctgcctgcccctcgtggggcgtcggctcctcagccccggctccggccgatccgtcccctccagggctatggggcccaaagggaaacatgatcaacgcccccgccccccgctccgggccactgccccgccggccgacacctcagtgcccctgttcagctgccacttccggcgtgcagcggcctaaccccac

SEQ ID NO: 15419 - RNA, 3961 nt, Homo sapiens
  source 1..3961: mol_type = other RNA
gctgggattacaggcatgagccactgcgcctggccgagtagagaagaatttactgctgattaaggttgtgtttttcaacctgcaatcccgagaccctcagaataaagattacttgaggttgctatgaaaaatacagattcctgtcctccccctggctgaatcagaatctcataaggtgaggctcaggtttctgcacttttcacaagctctgtaatggttacagtgcaccctaatgtttgagaaccagtggcctaaagagaatgcaacctaagagggcaaggctagtgcatagcttaaatcgctccagcctttggtaatcccttctaaacacagtaccacccatgtggaggagactgcaaggaagctgttattcaaagtagaacagtcagccttgtgcttgagtcctgctttatgcttgcgtgtttcataacaaaacacaaaggcaagtcttcatatcagcacttagtcttgatatccaagtagctgactactgtacttatgataacagcttgaagaggactgcaactctcccctcacgaatggtgacagagttggcttgtcacacctggctcagggaagaaaaatgagtaaacccctacctctttactcttgattcctcttccaccctaatactgttaacacatcatcctgtgtgattcaaataatctggcagatgaaatacagaaaatctaagtcatattgttcttatcactctatggccagatattatactaatctaattttaaaaatccttttctgtgcaatagaaataaccaaagctcattctgtctcctttcctttctaatgctgttgataggaacaaaatatcaagtaaggatacatgctagagatgttaaattcatacaagtaaagtaaattacaaagagaggtggtaatatttttttctagaatttcacaataaaatccctctcaccatgaaaatctttttataattttaacaggaaacttaaaagacattttgttgcaagactatcttaacaattataagaataatgccattatctgtgctcaatatagataaacataacagtaactttaaaaggccaagtatactcataagtgaggatgaaatttatttttcaacaaccaatatgccaatatccaacttctaggttttattcaattctaatgtcatgggtttctcctaccccagtcaaaactcctgccaaatgtccacaaaattgacaccaaaatcaacaaacacaaagaaagagagggacagggagagggaaagagaaatagagagtgaggaaggaaggaacgtgacaagagctaccatgcaaaatgaccagaagaactggagttcagtggcacagatcagcaggagcagaggaatgctgcaaaagatgatgctgcatagagtctaacttggagatgcctgtatgatgctggatgaccaagtactaaggtcacaagtgtgttcatggacccataagaaccaggatcttgacccaaacttataagatcttctaaaaagaaaatacttcatctaaattgaagcaattcctaagtcaaacaccagaagagttccttatttgatgtaagttgtgcctaaaactttggctgatacaaagaaacccgtccactaaggcaccctgaggcaatctgacaatgtgttggagagaactttgttgtcagtaccacatcattatgagagtacagagaacggatcacccgcaggggactggcttctttgggcaagcagtcaacaagttcactgcactgtttgtcaaatcccaacaagcgaatcccatagccatgtggggaagaaatcattcgtccatcggggctgaagcaaagttctttgatgtaacccctgcctacattggcttcttcaatgtaatgagtcagtcgtagagaacagcgaggtgagacaggtcgcactggagctccttcttggaattcatagacacaagtacactcttcccctacacaattcaaaggctcttctcttctctcctttcagttgtggcctctaggaccagtgagatccttggaagactcttgctttccagagtgatgagaatcataaagtcatttaacacctttccccctagtcatcagtatagtcccttcctttcccagagtttcccctggtttttaaaaaaagaaaattatgatactcaattggcttagtaaaatctcacatttagccagcttagctgaaacatttcagacctatgtttattatacaaggggtttttgtttgtttgtttgtttgtttgtttagggtgagatgaaagaggcaagatttaagaagctgggcaaaaactgagctgatgctggcctttaaagtacctcccaccttgctcaaccccagcaggagaggaataagaagagtttggaagggataatgataccatatgaagcaagagaggacagaaacaggagagtcgagaagcaggatctctagcagtatgcccttgaaggcagagactgcagtcagcgatcggcctaagctctgcacacacggcaatggcaatttgtccaatgagccctgttgaaggtggagtgctgctgcctgtacctcctcatcatcactgttgcttgagcaccgaagaagagtggcccagccttttgggtgcagctgtaaggacgtgatgcagtttccgtggtcactctcaccaagaacttcaggggttacgacttcaagactatttcgtggtgaaactccttctctttgagaggctcgtgacatgtgtttctcagaagaattagaatcactatgatgacaaggtgagccagaaactctaggaccagatgaacttgatgaagtggtcaaatctgaacttgaagtagttcttcttgctcttaaaatgggatagctgcctacttctaaagacttagttaagtcaaggtcatgcaaaattaagagatatccagaggacgttgaaatcaacattttggaacaatctggtgttaacctcattcgcatgagaaaacgtgtgtgaaagaatttcttatgtggacacccatcttctgtatacctgttagtgtcccaaataatgacatttccatcaaatcctgatgttactaagagtcttgtattagtatcatattcgatgttcttcacccagctagtgtgaccatgtaaagtgcatactttggtgttcaattttctcagatcccatagtgctattgtagtgtcatcagagcaggtagcaaacagccggttatcaagaaatctgatattatttacacagtcttcatgagcttcagaaagtgtttttatgtgctttgaagatatagggtcaaaaagcagaacttcagtttgttcacaagcaactgtcagcactgacccgtcgggcgagtactcgaggttgaagacggcgccgtgggtgcgggtgctgaggtacaccgagtccgcggggtggatggaaccgtagaggctagtcatggtgcgaaaattgtcccgcgccgggtccacgaacagcccgcggcccaggctgcgctctttcagccacccgaacagcctagcgccagggccgcccaggcccgcgccgaggccgtgtcggccccggctcttggccctgcagtctggcccgggccgccggcacggaggggagggaggtgacggctctcccggggcggaggcagttgaggactccggagctccaggcagccctagctctccggagcgcggggccggggacagcgatggggcgccggggcggcgagggcttcgggcgggtggagggggatgggtcgcatcagccccgggatgtagtggcgagggcggcccggtggctgctgcctgcccctcgtggggcgtcggctcctcagccccggctccggccgatccgtcccctccagggctatggggcccaaagggaaacatgatcaacgcccccgccccccgctccgggccactgccccgccggccgacacctcagtgcccctgttcagctgccacttccggcgtgcagcggcctaaccccac

SEQ ID NO: 15420 - RNA, 863 nt, Homo sapiens
  source 1..863: mol_type = other RNA
gctgggattacaggcatgagccactgcgcctggccggaaagatttccttaaaacaaaagtgcatggaattgctgttcttacatttgtttattgtgatatttcactgttgcataccctgataccaaattagtgtaagtactgtgtaagaaaaaaacaaacaaacatgtaactaaatacttttccataccgttttccaagtcaagaatgaccagaaaaagtaggtagtctctcatatttgtttagcatgtccactttttacttattgttaaattactcagtctcaaattgtacaatgcttgaaaacagatatgacaatttctgagattaaactttattaaagttacttttccagaaaattcagtaaatatggtaatataggaacaaacttaggctcataagccttttaactttttacataatctttaatgatgttgatcaggaaattctttcattggtggaattacttctccagtctccagaattgtatcaccagaaacatgatacttcatgtaataatgaataatccagacaggtacaagtacatgagtgaaaacaaagatactctttttgtataccccatggaccattttcctccaaggggatttattctccaaaaatttattccagaatttctccataggccccatcttctgtgggggcagcaccggctcccgagggctcagctcctggtccttcagccatcgccttctcagctctcgcagctgctgcagccgcagtttctcatccggagtgtaccccgtcatgtcgccgctggtaccaacgcaaaaggacacggcgcaccctcgaactacggactagttacttaagcgcgctcccgctctgcaaagcgaccttgcgggaac

SEQ ID NO: 15421 - RNA, 908 nt, Homo sapiens
  source 1..908: mol_type = other RNA
gctgggattacaggcatgagccactgcgcctggccggaaagatttccttaaaacaaaagtgcatggaattgctgttcttacatttgtttattgtgatatttcactgttgcataccctgataccaaattagtgtaagtactgtgtaagaaaaaaacaaacaaacatgtaactaaatacttttccataccgttttccaagtcaagaatgaccagaaaaagtaggtagtctctcatatttgtttagcatgtccactttttacttattgttaaattactcagtctcaaattgtacaatgcttgaaaacagatatgacaatttctgagattaaactttattaaagttacttttccagaaaattcagtaaatatggtaatataggaacaaacttaggctcataagccttttaactttttacataatctttaatgatgttgatcaggaaattctttcattggtggaattacttctccagtctccagaattgtatcaccagggaatattctggacttcttttcaactatgccatatggtttttcagaaacatgatacttcatgtaataatgaataatccagacaggtacaagtacatgagtgaaaacaaagatactctttttgtataccccatggaccattttcctccaaggggatttattctccaaaaatttattccagaatttctccataggccccatcttctgtgggggcagcaccggctcccgagggctcagctcctggtccttcagccatcgccttctcagctctcgcagctgctgcagccgcagtttctcatccggagtgtaccccgtcatgtcgccgctggtaccaacgcaaaaggacacggcgcaccctcgaactacggactagttacttaagcgcgctcccgctctgcaaagcgaccttgcgggaac

SEQ ID NO: 15422 - RNA, 815 nt, Homo sapiens
  source 1..815: mol_type = other RNA
gctgggattacaggcatgagccactgcgcctggccggaaagatttccttaaaacaaaagtgcatggaattgctgttcttacatttgtttattgtgatatttcactgttgcataccctgataccaaattagtgtaagtactgtgtaagaaaaaaacaaacaaacatgtaactaaatacttttccataccgttttccaagtcaagaatgaccagaaaaagtaggtagtctctcatatttgtttagcatgtccactttttacttattgttaaattactcagtctcaaattgtacaatgcttgaaaacagatatgacaatttctgagattaaactttattaaagttacttttccagaaaattcagtaaatatggtaatataggaacaaacttaggctcataagccttttaactttttacataatctttaatgatgttgatcaggaaattctttcattggtggaattacttctccagtctccagaattgtatcaccagggaatattctggacttcttttcaactatgccatatggtttttccattttcctccaaggggatttattctccaaaaatttattccagaatttctccataggccccatcttctgtgggggcagcaccggctcccgagggctcagctcctggtccttcagccatcgccttctcagctctcgcagctgctgcagccgcagtttctcatccggagtgtaccccgtcatgtcgccgctggtaccaacgcaaaaggacacggcgcaccctcgaactacggactagttacttaagcgcgctcccgctctgcaaagcgaccttgcgggaac

SEQ ID NO: 15423 - RNA, 6399 nt, Homo sapiens
  source 1..6399: mol_type = other RNA
gctgggattacaggcatgagccactgcgcctggcctacgaggtgacctttaacttgaaaacatggagttcttcaccaaaaaagtattcaaatgatagtttttaaacaaggaaatatggtctaaaaaagatacaacctgtcttccaatggcctttccattctagtgtttcctaatatattacactagaagttaactataaattatatactttaaaatataaagtattgattgtcagtataaggttcccaggccaggaaagaggaggggaaagtcctttgccaagaccctcccccaatttctttgtaagatgatttcacctttaaagaactcccagagagtaaagggcaaaaacacgtttacaaggaggccccaacattacaagtgcctgttttagaacagattgtgtcagaggtgtaagagatctagaaacttttccccacttaagaaaaaaaggcaagaaaattaagtatttgatacttaactgccctcttcatagaccactgtctggggatctattttctatgtacaggtttgccagctttaaaatactgaatgtcagttattcctactttggtatccaaaatatccataagcaatatatgagcatccattccactataatttctgaaaattcactaaaataagagcatttttaaaaattaactttaaaagatacatttgcatactttatttttgatggatttatttttaaatagctaaaaacataaagcaaattctttggagcccatggcaattactttttcccctgtccacttgagtgaaatgccatagagctaaagagaaaaactaaaccatttcttagattgaataaaagatcattaattgttgacacatatctaaatcatttcagtatatttagaaggcaaagaagaaagggagaaggaaagaaaagagagaagaaaagaaaaaagggggattcatctttaaaatttccatccagataaattatattacccttcggaatacagggcaattaaagattgaggtgctcaggattcggggatcttaaaagttcacagcaagcatcagatgtcactagacaactggcagtctaatgctcacacccctgaactagaagaggttccacaggatccctggccaatgccagggatctttaggtcagcagtcatgtcaagatgctctgattctccacaaacccagcttctttcccaaactgcagggaggtcggtctgcagtgacttacctagtattttgttgtatccctggctcacagtgtctccctggtctaggatcttcgaatcgaaatcccatgaagcacatattgcagtgctctctgactctcacccctgaaatagagctggtgtggggctgaggatgtgggaaggagacagcacacccagcaccccccagggcaattttcagtatgctcctcaacctctgagatggtgtgaaaagcacagtaaatgtactgcccctcacatttctctacagaggaaaaagagagggagggcaatggctggggggtgtgatcagatttcaagcagaaaaagaccgtgccacttaaaaaaaattcaccacctagattctgaaaagaaagaatttccagttaagaagtatctactgagaccactgggcatggggtgggttggggtggggtgggcagtagggctaggttggaggtgggaagggaacagatgaagctcctcctgctggctgttttctcccattcccagggaaatccatctttaagcaaacatggatgtgtaataatgcttaagaatctaggttcatttctttcacaaaatgaggagaatacctattctaaagtaatacctttattctggagaaaacaaacacctccaaaaaaattctaaaagattttgagaggggaaaatatagacacacaactgcattcattctgatcttccacacaaagatcaggtgaagaaatctatgcagctatacatgctaggacctgttgtacaccatccctgcaaccccatagaaagaaaaaaaactcttttttcaaaatagaagcagtattcttctacgaaaacaaaacaatcacatgtgactactggaaatgttagtgttacacagagtcctttaaaaataaatcacagccaaagttccataaagtacagaagcttgaaacagaaaataaaaatgactgaagagtgatgatgggagcctgaagctccatcctcacaaggacggcagccctggacatcactgcaaaggtcacaggaggacagcttcacttcagagttgtaacttctcaccgcctgtctccttggctcatagtaatccactatggacactgaagcatcttgggtatttgaaactttaaagtttctcacagcaggaatattaacacaaaactgggtttcatttacagaatctaaatagaggttgagttttccatgatcatattccactttcttcactgtctcgctcagagaaattgcttctgaaggcaccataaagccacttaataggttaacttccataagagccatgccactcctacccgggcccgaaaagcttgtacacacattcaaatccacatgattgagatcatctttattttcttttacagcaacatctaaatcaaaggcttcttgattttggatagatcttcgtcttctagaagacccagaagccttcacattatatacaacattgagctgacaaatagcaaatccaaaaccatttgcggaaatattaactgccgttggctgtaccacagcaagaggacttggtgagctaggccccgtcacggtcacttggatatttgtcctttctgtattcattagggctgcaaattcagacagagcctttaaagccacagtggtatcctgagtagatgcaaaaccacccaagctatttctttgcctgcttagccacctcataattgggattccctcagaagtctgaaattgtaagaagtgtgagagcagtgcataggctgcaacttcaatatccagggagcgtggctgccaggagtcagaaagtttggactctgatgacacccagaattgcatgccaccttcttgttctgctctccaagtcagcatattcaaagcttccttcgctttaggactccccactgatgacaatgcataagttataagggctagagtataattgtctgaaattcctctactgaattcagactccaaaaaatggatagactcttgcacatcaatgttaggctgatactttctatatcccaggagagaagttacaatataggctgtaagtgttactggacttttattgccaccttgaagctcactatgaatcactcttcctggatcccaaaattcaccgttggatttctgatgtcctttaagccaagtgtatgttctgtgtaacacattctgatcaatatctatgtaaggatcggcttcaaggaaacatcttaaaacaaaagctgacaaccaagtgctcccagaagggtcataattcccaaaagcactgaaagagccatcttccctctgatagagaagttctctctggtaaccttgcctcataaatgaaagagctttttctttcaaattatctgtcagttgtttctttttagtcagataatccaaaatgtaaatatttggagcaaaatttatcatgttctgttcaccacagccataaggcatccgaatcaatgaggctaagccattgatggaaggaccaagaacatctccaattgcagtgatctgaactctttcactgccagtcactgtattaggaggaaatgagaaactcaaagttttcagggtactctgtagcctattgtcagtcaagtctaataagatggattgtgaatatgatttttctattccttcagcctttactaaaatcatctgggtgacagcatcagaagcagtgggtgaaagagctgtgactgtgataggaatttctcccagatgtgttggcctgatgggaaaaagaacagttgccccatcctcactgggaaccagaagggtctgctggtggcctgtggcatttatttcatttgaagtcattagaatatcaaatttgtcacttttctcaatgattaccttaacctcagtggcatctttcaaataattgaatatagttatttccaaagcaaattcttcacctctgataacagagtagggaagattcaaaaaaatgaaaaatggttggaaggcttggagctccactggagtagttgttagtccaagacccaggtcctcagagatcacaaaaccagtagccacccaagaagtgatagaatcaggtacagttacttcaaattcttggtaaatcctgtaacccatgttggtgtctagccaaatccaagtctctggaaaatgctttcggacatgtggactgctacccaaagaaaagtcatgaatatctacaatatgtccttcattttcctccataaacctctcagcatattctgcattgtcataaacaccatcaatataatccttcgtgaggtttgcatctgtcaatacccagagtccacattcctgaaagactgcaaaagaattcatgaacatgcctaaataatatcctgtgttataaagttccaactcatggaccacattttccattgtaatatcattagaggcattcatcagattcacacttttgtcaacagctacaatcccaactatggagtcaggctgtgtcacagagatcctaagagagactttctcagatggttcagctttcactttactccaatatagctttatcttatttttaaaaacaagctgaacaggaatttttagaacatcacttataatttccccatcatcttcaatataatacacaattacacaggcttttggagtccaagaattttctggtgttaaagagaacattgttgaattttgttttcctacagccaccaactgtcccctggatactaccatatagcttaactccttcaatcgtttgttgccactaaccaccaactcaaaaggcgatcccacctttatattttcatctcttgtttttagttggatgtatgtcttactaggagacttaaacagactatgaactgccatgctacttttactaccaaggaaataggccttcaactgtagctcactggaatcctccaggattgggaattcaatcttaaaagttccactttgggggacagtataatttattttctgaacagcttccattttctgatttccactgttagatccgctccagtactcagtatagtttctctgtgtcactgttatgactacattatttcttctttcttcaagagtcagttggttgccatcagcacgagttaccttcacagtggctgtgaagttgagagatggcttcaagacagtagtataatcaaaaaactcaatgatgtaatcatgttgcttgaagaacacattagtgcttacatttcttgaaatacctgtaactgattctgtcactgtggttaaaatttctactggtccaggggaagatagatccaggtattcagaaagtccatttgaagaatccattacatttttcatctcttcatcattaaaagagaagtttgcagatccatttatcttaaatgtttttgtaatatttttcttctttccccaaaaggataaaggtaaaaatgtaagcgttacgtctcctttcactggcttcccatatgtatactttgccgtgatggtaccatttaaatgcttagaattcatagaacaatataatggtgtctgcaaagtcacttcaaattttggtaatacatattctgaaacctgaaatgattgatagtatgtctggtcattcacttgaacttgaatagaccagtcaccaagtattggatgggaagatagctgaaaagttttggaaatgactccaagatcactttgttgtgacaaccactgttggatcaaatttgatttggggtccttaatgagaatgtttaaagaggttttgtaaggcttaaaatctgagaagagtgtaacaatgcgaaacttcacttcttgctttggcttgtataaggccttgtctgtttgaatgaagacagatattctcttggtctcaaatgataagcgggtactattagagaataaaatctcatcctgggtacgtccggttacacgtagctcataaatctcatctgcactgttcagaggtagtgatggaagagtaagtgtcttaaaagagcctttttcaaagactccttctgcttccaggacagagacagtgaggtttgatgctgtcttgagcagctccgccttcacagtcacctgtgaagggcagtgttccagaagctccaccccaatagtcacatttcctccgggcctgatgatccctggggctgtcaccagaaaccgaggcccgggagccacggccagcgcggcggtgcacacgcagaggaggtgggcggcggtcaggagcggtgggccctgcatctcgacggcgtct

SEQ ID NO: 15424 - RNA, 6450 nt, Homo sapiens
  source 1..6450: mol_type = other RNA
gctgggattacaggcatgagccactgcgcctggcctacgaggtgacctttaacttgaaaacatggagttcttcaccaaaaaagtattcaaatgatagtttttaaacaaggaaatatggtctaaaaaagatacaacctgtcttccaatggcctttccattctagtgtttcctaatatattacactagaagttaactataaattatatactttaaaatataaagtattgattgtcagtataaggttcccaggccaggaaagaggaggggaaagtcctttgccaagaccctcccccaatttctttgtaagatgatttcacctttaaagaactcccagagagtaaagggcaaaaacacgtttacaaggaggccccaacattacaagtgcctgttttagaacagattgtgtcagaggtgtaagagatctagaaacttttccccacttaagaaaaaaaggcaagaaaattaagtatttgatacttaactgccctcttcatagaccactgtctggggatctattttctatgtacaggtttgccagctttaaaatactgaatgtcagttattcctactttggtatccaaaatatccataagcaatatatgagcatccattccactataatttctgaaaattcactaaaataagagcatttttaaaaattaactttaaaagatacatttgcatactttatttttgatggatttatttttaaatagctaaaaacataaagcaaattctttggagcccatggcaattactttttcccctgtccacttgagtgaaatgccatagagctaaagagaaaaactaaaccatttcttagattgaataaaagatcattaattgttgacacatatctaaatcatttcagtatatttagaaggcaaagaagaaagggagaaggaaagaaaagagagaagaaaagaaaaaagggggattcatctttaaaatttccatccagataaattatattacccttcggaatacagggcaattaaagattgaggtgctcaggattcggggatcttaaaagttcacagcaagcatcagatgtcactagacaactggcagtctaatgctcacacccctgaactagaagaggttccacaggatccctggccaatgccagggatctttaggtcagcagtcatgtcaagatgctctgattctccacaaacccagcttctttcccaaactgcagggaggtcggtctgcagtgacttacctagtattttgttgtatccctggctcacagtgtctccctggtctaggatcttcgaatcgaaatcccatgaagcacatattgcagtgctctctgactctcacccctgaaatagagctggtgtggggctgaggatgtgggaaggagacagcacacccagcaccccccagggcaattttcagtatgctcctcaacctctgagatggtgtgaaaagcacagtaaatgtactgcccctcacatttctctacagaggaaaaagagagggagggcaatggctggggggtgtgatcagatttcaagcagaaaaagaccgtgccacttaaaaaaaattcaccacctagattctgaaaagaaagaatttccagttaagaagtatctactgagaccactgggcatggggtgggttggggtggggtgggcagtagggctaggttggaggtgggaagggaacagatgaagctcctcctgctggctgttttctcccattcccagggaaatccatctttaagcaaacatggatgtgtaataatgcttaagaatctaggttcatttctttcacaaaatgaggagaatacctattctaaagtaatacctttattctggagaaaacaaacacctccaaaaaaattctaaaagattttgagaggggaaaatatagacacacaactgcattcattctgatcttccacacaaagatcaggtgaagaaatctatgcagctatacatgctaggacctgttgtacaccatccctgcaaccccatagaaagaaaaaaaactcttttttcaaaatagaagcagtattcttctacgaaaacaaaacaatcacatgtgactactggaaatgttagtgttacacagagtcctttaaaaataaatcacagccaaagttccataaagtacagaagcttgaaacagaaaataaaaatgactgaagagtgatgatgggagcctgaagctccatcctcacaaggacggcagccctggacatcactgcaaaggtcacaggaggacagcttcacttcagagttgtaacttctcaccgcctgtctccttggctcatagtaatccactatggacactgaagcatcttgggtatttgaaactttaaagtttctcacagcaggaatattaacacaaaactgggtttcatttacagaatctaaatagaggttgagttttccatgatcatattccactttcttcactgtctcgctcagagaaattgcttctgaaggcaccataaagccacttaataggttaacttccataagagccatgccactcctacccgggcccgaaaagcttgtacacacattcaaatccacatgattgagatcatctttattttcttttacagcaacatctaaatcaaaggcttcttgattttggatagatcttcgtcttctagaagacccagaagccttcacattatatacaacattgagctgacaaatagcaaatccaaaaccatttgcggaaatattaactgccgttggctgtaccacagcaagctctgctgtctgaaggagtaagcggttgtgtgtgtcaatcagaaactttacaggacttggtgagctaggccccgtcacggtcacttggatatttgtcctttctgtattcattagggctgcaaattcagacagagcctttaaagccacagtggtatcctgagtagatgcaaaaccacccaagctatttctttgcctgcttagccacctcataattgggattccctcagaagtctgaaattgtaagaagtgtgagagcagtgcataggctgcaacttcaatatccagggagcgtggctgccaggagtcagaaagtttggactctgatgacacccagaattgcatgccaccttcttgttctgctctccaagtcagcatattcaaagcttccttcgctttaggactccccactgatgacaatgcataagttataagggctagagtataattgtctgaaattcctctactgaattcagactccaaaaaatggatagactcttgcacatcaatgttaggctgatactttctatatcccaggagagaagttacaatataggctgtaagtgttactggacttttattgccaccttgaagctcactatgaatcactcttcctggatcccaaaattcaccgttggatttctgatgtcctttaagccaagtgtatgttctgtgtaacacattctgatcaatatctatgtaaggatcggcttcaaggaaacatcttaaaacaaaagctgacaaccaagtgctcccagaagggtcataattcccaaaagcactgaaagagccatcttccctctgatagagaagttctctctggtaaccttgcctcataaatgaaagagctttttctttcaaattatctgtcagttgtttctttttagtcagataatccaaaatgtaaatatttggagcaaaatttatcatgttctgttcaccacagccataaggcatccgaatcaatgaggctaagccattgatggaaggaccaagaacatctccaattgcagtgatctgaactctttcactgccagtcactgtattaggaggaaatgagaaactcaaagttttcagggtactctgtagcctattgtcagtcaagtctaataagatggattgtgaatatgatttttctattccttcagcctttactaaaatcatctgggtgacagcatcagaagcagtgggtgaaagagctgtgactgtgataggaatttctcccagatgtgttggcctgatgggaaaaagaacagttgccccatcctcactgggaaccagaagggtctgctggtggcctgtggcatttatttcatttgaagtcattagaatatcaaatttgtcacttttctcaatgattaccttaacctcagtggcatctttcaaataattgaatatagttatttccaaagcaaattcttcacctctgataacagagtagggaagattcaaaaaaatgaaaaatggttggaaggcttggagctccactggagtagttgttagtccaagacccaggtcctcagagatcacaaaaccagtagccacccaagaagtgatagaatcaggtacagttacttcaaattcttggtaaatcctgtaacccatgttggtgtctagccaaatccaagtctctggaaaatgctttcggacatgtggactgctacccaaagaaaagtcatgaatatctacaatatgtccttcattttcctccataaacctctcagcatattctgcattgtcataaacaccatcaatataatccttcgtgaggtttgcatctgtcaatacccagagtccacattcctgaaagactgcaaaagaattcatgaacatgcctaaataatatcctgtgttataaagttccaactcatggaccacattttccattgtaatatcattagaggcattcatcagattcacacttttgtcaacagctacaatcccaactatggagtcaggctgtgtcacagagatcctaagagagactttctcagatggttcagctttcactttactccaatatagctttatcttatttttaaaaacaagctgaacaggaatttttagaacatcacttataatttccccatcatcttcaatataatacacaattacacaggcttttggagtccaagaattttctggtgttaaagagaacattgttgaattttgttttcctacagccaccaactgtcccctggatactaccatatagcttaactccttcaatcgtttgttgccactaaccaccaactcaaaaggcgatcccacctttatattttcatctcttgtttttagttggatgtatgtcttactaggagacttaaacagactatgaactgccatgctacttttactaccaaggaaataggccttcaactgtagctcactggaatcctccaggattgggaattcaatcttaaaagttccactttgggggacagtataatttattttctgaacagcttccattttctgatttccactgttagatccgctccagtactcagtatagtttctctgtgtcactgttatgactacattatttcttctttcttcaagagtcagttggttgccatcagcacgagttaccttcacagtggctgtgaagttgagagatggcttcaagacagtagtataatcaaaaaactcaatgatgtaatcatgttgcttgaagaacacattagtgcttacatttcttgaaatacctgtaactgattctgtcactgtggttaaaatttctactggtccaggggaagatagatccaggtattcagaaagtccatttgaagaatccattacatttttcatctcttcatcattaaaagagaagtttgcagatccatttatcttaaatgtttttgtaatatttttcttctttccccaaaaggataaaggtaaaaatgtaagcgttacgtctcctttcactggcttcccatatgtatactttgccgtgatggtaccatttaaatgcttagaattcatagaacaatataatggtgtctgcaaagtcacttcaaattttggtaatacatattctgaaacctgaaatgattgatagtatgtctggtcattcacttgaacttgaatagaccagtcaccaagtattggatgggaagatagctgaaaagttttggaaatgactccaagatcactttgttgtgacaaccactgttggatcaaatttgatttggggtccttaatgagaatgtttaaagaggttttgtaaggcttaaaatctgagaagagtgtaacaatgcgaaacttcacttcttgctttggcttgtataaggccttgtctgtttgaatgaagacagatattctcttggtctcaaatgataagcgggtactattagagaataaaatctcatcctgggtacgtccggttacacgtagctcataaatctcatctgcactgttcagaggtagtgatggaagagtaagtgtcttaaaagagcctttttcaaagactccttctgcttccaggacagagacagtgaggtttgatgctgtcttgagcagctccgccttcacagtcacctgtgaagggcagtgttccagaagctccaccccaatagtcacatttcctccgggcctgatgatccctggggctgtcaccagaaaccgaggcccgggagccacggccagcgcggcggtgcacacgcagaggaggtgggcggcggtcaggagcggtgggccctgcatctcgacggcgtct

SEQ ID NO: 15425 - RNA, 6219 nt, Homo sapiens
  source 1..6219: mol_type = other RNA
gctgggattacaggcatgagccactgcgcctggcctacgaggtgacctttaacttgaaaacatggagttcttcaccaaaaaagtattcaaatgatagtttttaaacaaggaaatatggtctaaaaaagatacaacctgtcttccaatggcctttccattctagtgtttcctaatatattacactagaagttaactataaattatatactttaaaatataaagtattgattgtcagtataaggttcccaggccaggaaagaggaggggaaagtcctttgccaagaccctcccccaatttctttgtaagatgatttcacctttaaagaactcccagagagtaaagggcaaaaacacgtttacaaggaggccccaacattacaagtgcctgttttagaacagattgtgtcagaggtgtaagagatctagaaacttttccccacttaagaaaaaaaggcaagaaaattaagtatttgatacttaactgccctcttcatagaccactgtctggggatctattttctatgtacaggtttgccagctttaaaatactgaatgtcagttattcctactttggtatccaaaatatccataagcaatatatgagcatccattccactataatttctgaaaattcactaaaataagagcatttttaaaaattaactttaaaagatacatttgcatactttatttttgatggatttatttttaaatagctaaaaacataaagcaaattctttggagcccatggcaattactttttcccctgtccacttgagtgaaatgccatagagctaaagagaaaaactaaaccatttcttagattgaataaaagatcattaattgttgacacatatctaaatcatttcagtatatttagaaggcaaagaagaaagggagaaggaaagaaaagagagaagaaaagaaaaaagggggattcatctttaaaatttccatccagataaattatattacccttcggaatacagggcaattaaagattgaggtgctcaggattcggggatcttaaaagttcacagcaagcatcagatgtcactagacaactggcagtctaatgctcacacccctgaactagaagaggttccacaggatccctggccaatgccagggatctttaggtcagcagtcatgtcaagatgctctgattctccacaaacccagcttctttcccaaactgcagggaggtcggtctgcagtgacttacctagtattttgttgtatccctggctcacagtgtctccctggtctaggatcttcgaatcgaaatcccatgaagcacatattgcagtgctctctgactctcacccctgaaatagagctggtgtggggctgaggatgtgggaaggagacagcacacccagcaccccccagggcaattttcagtatgctcctcaacctctgagatggtgtgaaaagcacagtaaatgtactgcccctcacatttctctacagaggaaaaagagagggagggcaatggctggggggtgtgatcagatttcaagcagaaaaagaccgtgccacttaaaaaaaattcaccacctagattctgaaaagaaagaatttccagttaagaagtatctactgagaccactgggcatggggtgggttggggtggggtgggcagtagggctaggttggaggtgggaagggaacagatgaagctcctcctgctggctgttttctcccattcccagggaaatccatctttaagcaaacatggatgtgtaataatgcttaagaatctaggttcatttctttcacaaaatgaggagaatacctattctaaagtaatacctttattctggagaaaacaaacacctccaaaaaaattctaaaagattttgagaggggaaaatatagacacacaactgcattcattctgatcttccacacaaagatcaggtgaagaaatctatgcagctatacatgctaggacctgttgtacaccatccctgcaaccccatagaaagaaaaaaaactcttttttcaaaatagaagcagtattcttctacgaaaacaaaacaatcacatgtgactactggaaatgttagtgttacacagagtcctttaaaaataaatcacagccaaagttccataaagtacagaagcttgaaacagaaaataaaaatgactgaagagtgatgatgggagcctgaagctccatcctcacaaggacggcagccctggacatcactgcaaaggtcacaggaggacagcttcacttcagagttgtaacttctcaccgcctgtctccttggctcatagtaatccactatggacactgaagcatcttgggtatttgaaactttaaagtttctcacagcaggaatattaacacaaaactgggtttcatttacagaatctaaatagaggttgagttttccatgatcatattccactttcttcactgtctcgctcagagaaattgcttctgaaggcaccataaagccacttaataggttaacttccataagagccatgccactcctacccgggcccgaaaagcttgtacacacattcaaatccacatgattgagatcatctttattttcttttacagcaacatctaaatcaaaggcttcttgattttggatagatcttcgtcttctagaagacccagaagccttcacattatatacaacattgagctgacaaatagcaaatccaaaaccatttgcggaaatattaactgccgttggctgtaccacagcaagctctgctgtctgaaggagtaagcggttgtgtgtgtcaatcagaaactttacaggacttggtgagctaggccccgtcacggtcacttggatatttgtcctttctgtattcattagggctgcaaattcagacagagcctttaaagccacagtggtatcctgagtagatgcaaaaccacccaagctatttctttgcctgcttagccacctcataattgggattccctcagaagtctgaaattgtaagaagtgtgagagcagtgcataggctgcaacttcaatatccagggagcgtggctgccaggagtcagaaagtttggactctgatgacacccagaattgcatgccaccttcttgttctgctctccaagtcagcatattcaaagcttccttcgctttaggactccccactgatgacaatgcataagttataagggctagagtataattgtctgaaattcctctactgaattcagactccaaaaaatggatagactcttgcacatcaatgttaggctgatactttctatatcccaggagagaagttacaatataggctgtaagtgttactggacttttattgccaccttgaagctcactatgaatcactcttcctggatcccaaaattcaccgttggatttctgatgtcctttaagccaagtgtatgttctgtgtaacacattctgatcaatatctatgtaaggatcggcttcaaggaaacatcttaaaacaaaagctgacaaccaagtgctcccagaagggtcataattcccaaaagcactgaaagagccatcttccctctgatagagaagttctctctggtaaccttgcctcataaatgaaagagctttttctttcaaattatctgtcagttgtttctttttagtcagataatccaaaatgtaaatatttggagcaaaatttatcatgttctgttcaccacagccataaggcatccgaatcaatgaggctaagccattgatggaaggaccaagaacatctccaattgcagtgatctgaactctttcactgccagtcactgtattaggaggaaatgagaaactcaaagttttcagggtactctgtagcctattgtcagtcaagtctaataagatggattgtgaatatgatttttctattccttcagcctttactaaaatcatctgggtgacagcatcagaagcagtgggtgaaagagctgtgactgtgataggaatttctcccagatgtgttggcctgatgggaaaaagaacagttgccccatcctcactgggaaccagaagggtctgctggtggcctgtggcatttatttcatttgaagtcattagaatatcaaatttgtcacttttctcaatgattaccttaacctcagtggcatctttcaaataattgaatatagttatttccaaagcaaattcttcacctctgataacagagtagggaagattcaaaaaaatgaaaaatggttggaaggcttggagctccactggagtagttgttagtccaagacccaggtcctcagagatcacaaaaccagtagccacccaagaagtgatagaatcaggtacagttacttcaaattcttggtaaatcctgtaacccatgttggtgtctagccaaatccaagtctctggaaaatgctttcggacatgtggactgctacccaaagaaaagtcatgaatatctacaatatgtccttcattttcctccataaacctctcagcatattctgcattgtcataaacaccatcaatataatccttcgtgaggtttgcatctgtcaatacccagagtccacattcctgaaagactgcaaaagaattcatgaacatgcctaaataatatcctgtgttataaagttccaactcatggaccacattttccattgtaatatcattagaggcattcatcagattcacacttttgtcaacagctacaatcccaactatggagtcaggctgtgtcacagagatcctaagagagactttctcagatggttcagctttcactttactccaatatagctttatcttatttttaaaaacaagctgaacaggaatttttagaacatcacttataatttccccatcatcttcaatataatacacaattacacaggcttttggagtccaagaattttctggtgttaaagagaacattgttgaattttgttttcctacagccaccaactgtcccctggatactaccatatagcttaactccttcaatcgtttgttgccactaaccaccaactcaaaaggcgatcccacctttatattttcatctcttgtttttagttggatgtatgtcttactaggagacttaaacagactatgaactgccatgctacttttactaccaaggaaataggccttcaactgtagctcactggaatcctccaggattgggaattcaatcttaaaagttccactttgggggacagtataatttattttctgaacagcttccattttctgatttccactgttagatccgctccagtactcagtatagtttctctgtgtcactgttatgactacattatttcttctttcttcaagagtcagttggttgccatcagcacgagttaccttcacagtggctgtgaagttgagagatggcttcaagacagtagtataatcaaaaaactcaatgatgtaatcatgttgcttgaagaacacattagtgcttacatttcttgaaatacctgtaactgattctgtcactgtggttaaaatttctactggtccaggggaagatagatccaggtattcagaaagtccatttgaagaatccattacatttttcatctcttcatcattaaaagagaagtttgcagatccatttatcttaaatgtttttgtaatatttttcttctttccccaaaaggataaaggtaaaaatgtaagcgttacgtctcctttcactggcttcccatatgtatactttgccgtgatggtaccatttaaatgcttagaattcatagaacaatataatggtgtctgcaaagtcacttcaaattttggtaatacatattctgaaacctgaaatgattgatagtatgtctggtcattcacttgaacttgaatagaccagtcaccaagtattggatgggaagatagctgaaaagttttggaaatgactccaagatcactttgttgtgacaaccactgttggatcaaatttgatttggggtctgatggaagagtaagtgtcttaaaagagcctttttcaaagactccttctgcttccaggacagagacagtgaggtttgatgctgtcttgagcagctccgccttcacagtcacctgtgaagggcagtgttccagaagctccaccccaatagtcacatttcctccgggcctgatgatccctggggctgtcaccagaaaccgaggcccgggagccacggccagcgcggcggtgcacacgcagaggaggtgggcggcggtcaggagcggtgggccctgcatctcgacggcgtct

SEQ ID NO: 15426 - RNA, 1070 nt, Homo sapiens
  source 1..1070: mol_type = other RNA
gctgggattacaggcatgagccactgcgcctggcctcttcattgtctctttaatcatcatttcttcagggttcactaagttcctcagtcaggtacaaaggtggagtcatcctgattatcttctgcagaaagaggctggacttgcttgggttggttattactcaatgttttcttttgcctttccattatttctgttgtaaaaaatctctgcaagatccaatctagaagtgcccatgggttccaaattgtaggattcgaatctgatgttaaaagctgtgtccttcactctttgcagtcccattagaataattgtgatcctccctgagacagctgaatactgtggacaacgtgggtggtagtggttgcgggaggtaagtgggaaatcatgcacctttcagatcttagctcgaacatcagctgctcagggcggccatccctgcccatgcgtcctctccgtctgtcctctctcaggagcacttgttatactctcagggtccccccttttttttttaatgctttgcacaaattgtttccttgcatttctgtgtgccagatctatgcagacactgatcctaagagtagcttgaggatatcttgtttcttgactttacttcttcccttggaaacaggcatcatataggacctcacagggaatgaatagagagtgaaatcctccaaagcatacaaaacctaagaatacggactcctatgtgaaaaccttctgatgtaaaatgaagtaaaatgagataacaatctaaaaatgtttcagaagaaagggaaaaaaatataccataagaaagcacagtttttgccaggtgcggtggctcacgcctgtaatcttagcaggttgggaggccaaggcgggcggatcacttgagatcaggagttcaaaaccagcctggccaacatggtgaaacctcgtctctactaaaaacacaaaaaattagcagggcgtggttgggcacctgtaatcccagctacttgggaggctgaggtaggagaattgcttgaaccgggagtcagaggttgcagtgagccaagatcgtgccactgcactccagcctgggcaac

SEQ ID NO: 15427 - RNA, 1599 nt, Homo sapiens
  source 1..1599: mol_type = other RNA
gctgggattacaggcatgagccactgcgcctggcctctttgaatttttttaaaaacatcctggtgctaaaaggcagcaagattcataaatgcaaacaaacatataaataaacaaccaggccctcttcccttttaaataatctgtgaaataaaaataatctatctgcataggaaacaattatcaaatcagcatctacaatgtggcccaataaaagaaagggttttcatatttgatcctgtttttggttcctcaaaattaaaaacttggctccactctgtgctgtataatgatagattttttttaagaagagagagagtgggaattctcttgctgtttccatgggtttcatcatctttttttccatgactcataatggcttcttgcaaacactcttgttcccttgatctcatggagcgaatgaatgctcttaagctagttttcatcaaccagtcagcattcctcctgctttccaactgtgcatcctcagctggacacaaacattttccagtctactcattcacaaaataaacttctgagtattcttcaaagggctcggtccaacttgcccggggatattcgtgtatattgatctcactgatgcactgtggaagtaacttatagttctggaattgggggaagcacttcctggacttgatccaaaggcagcctctgcgtggtctctgaaagaacctgcacattcaatgctctcagtttctccgaatcacttcctcttaagagaacagatgtaggtttgtctctatgactctgccacttttgcactcttctctggccttcaagtattttgcggatagtgaggatgatcaaaaatataaaaactaatagaactaaaatataccaagtgatcttcatggaacaagtgatattttttatatccatctctaggtgcaaagaaatgtgtatacaatcattcgggtattccatgattctacaagtgtagtttatcgatttctccttgcttggctcatcctccatgattgttgatcttccagtgtggttttttagatgacaggtagtgttatattcctccaagtggtcaaccagaggagctacactgaagttaaagtgctgacaaggtgaatgaaaatcatttgctttcacttccattgatcctctcctgataagaacttttgatgtttgttcctgagaaataaaatccatgtttcctttagactcacaaaccaaacacgaggagcacattttaaattcacctgtgatgtcttggcaagtcctggtgaagttacgaaaattggagggatttagaaagattctcatgataatctgagtttcccttactggttgcagaaaagtcacaaaagaaaaatttaaggaggagagtgaataggtaaaattagattgcaaacacacttccagacatgatagctccaatgttctttctttcggtgtcttgaaatattccggcaaaattaaaatgaatgtgatcactattgccacaaataatttaaggagggctgtttttgtcatgtctcttcacatgacacaaatgtgttcccttgcagtacattcatggtatgttgcttcctgctttaagtttatctctgcagcactttaggttaatgc

SEQ ID NO: 15428 - RNA, 1579 nt, Homo sapiens
  source 1..1579: mol_type = other RNA
gctgggattacaggcatgagccactgcgcctggcctctttgaatttttttaaaaacatcctggtgctaaaaggcagcaagattcataaatgcaaacaaacatataaataaacaaccaggccctcttcccttttaaataatctgtgaaataaaaataatctatctgcataggaaacaattatcaaatcagcatctacaatgtggcccaataaaagaaagggttttcatatttgatcctgtttttggttcctcaaaattaaaaacttggctccactctgtgctgtataatgatagattttttttaagaagagagagagtgggaattctcttgctgtttccatgggtttcatcatctttttttccatgactcataatggcttcttgcaaacactcttgttcccttgatctcatggagcgaatgaatgctcttaagctagttttcatcaaccagtcagcattcctcctgctttccaactgtgcatcctcagctggacacaaacattttccagtctactcattcacaaaataaacttctgagtattcttcaaagggctcggtccaacttgcccggggatattcgtgtatattgatctcactgatgcactgtggaagtaacttatagttctggaattgggggaagcacttcctggacttgatccaaaggcagcctctgcgtggtctctgctgaaagaacctgcacattcaatgctctcagtttctccgaatcacttcctcttaagagaacagatgtaggtttgtctctatgactctgccacttttgcactcttctctggccttcaagtattttgcggatagtgaggatgatcaaaaatataaaaactaatagaactaaaatataccaagtgatcttcatggaacaagtgatattttttatatccatctctaggtgcaaagaaatgtgtatacaatcattcgggtattccatgattctacaagtgtagtttatcgatttctccttgcttggctcatcctccatgattgttgatcttccagtgtggttttttagatgacaggtagtgttatattcctccaagtggtcaaccagaggagctacactgaagttaaagtgctgacaaggtgaatgaaaatcatttgctttcacttccattgatcctctcctgataagaactgtgatgtcttggcaagtcctggtgaagttacgaaaattggagggatttagaaagattctcatgataatctgagtttcccttactggttgcagaaaagtcacaaaagaaaaatttaaggaggagagtgaataggtaaaattagattgcaaacacacttccagacatgatagctccaatgttctttctttcggtgtcttgaaatattccggcaaaattaaaatgaatgtgatcactattgccacaaataatttaaggagggctgtttttgtcatgtctcttcacatgacacaaatgtgttcccttgcagtacattcatggtatgttgcttcctgctttaagtttatctctgcagcactttaggttaatgcagttcacctcatactcacttccttttgagtaagaaaaaataaaacggtgggctgggcgaag

SEQ ID NO: 15429 - RNA, 1877 nt, Homo sapiens
  source 1..1877: mol_type = other RNA
gctgggattacaggcatgagccactgcgcctggcctctttgaatttttttaaaaacatcctggtgctaaaaggcagcaagattcataaatgcaaacaaacatataaataaacaaccaggccctcttcccttttaaataatctgtgaaataaaaataatctatctgcataggaaacaattatcaaatcagcatctacaatgtggcccaataaaagaaagggttttcatatttgatcctgtttttggttcctcaaaattaaaaacttggctccactctgtgctgtataatgatagattttttttaagaagagagagagtgggaattctcttgctgtttccatgggtttcatcatctttttttccatgactcataatggcttcttgcaaacactcttgttcccttgatctcatggagcgaatgaatgctcttaagctagttttcatcaaccagtcagcattcctcctgctttccaactgtgcatcctcagctggacacaaacattttccagtctactcattcacaaaataaacttctgagtattcttcaaagggctcggtccaacttgcccggggatattcgtgtatattgatctcactgatgcactgtggaagtaacttatagttctggaattgggggaagcacttcctggacttgatccaaaggcagcctctgcgtggtctctgctgaaagaacctgcacattcaatgctctcagtttctccgaatcacttcctcttaagagaacagatgtaggtttgtctctatgactctgccacttttgcactcttctctggccttcaagtattttgcggatagtgaggatgatcaaaaatataaaaactaatagaactaaaatataccaagtgatcttcatggaacaagtgatattttttatatccatctctaggtgcaaagaaatgtgtatacaatcattcgggtattccatgattctacaagtgtagtttatcgatttctccttgcttggctcatcctccatgattgttgatcttccagtgtggttttttagatgacaggtagtgttatattcctccaagtggtcaaccagaggagctacactgaagttaaagtgctgacaaggtgaatgaaaatcatttgctttcacttccattgatcctctcctgataagaacttttgatgtttgttcctgagaaataaaatccatgtttcctttagactcacaaaccaaacacgaggagcacattttaaattcacctgtgatgtcttggcaagtcctggtgaagttacgaaaattggagggatttagaaagattctcatgataatctgagtttcccttactggttgcagaaaagtcacaaaagaaaaatttaaggaggagagtgaataggtaaaattagattgcaaacacacttccagacatgatagctccaatgttctttcatagcaatatttgaaaggcaggtttgagacataggagactgctcattttacttgtcaaaataagagaagcaaatgaatattatgaaattccctgtagataaagaaaatggcaggaaaatgactcagggtaaaaagacacatacctttcaagtaaaatattctgcaaaataaatttcacacgctagcacaacttaaaatctctaggtttgtgatgaaatttaatctttcaaaaatatgaggataacacttggcctgcctaaatcacaagatgtttgtgaacgtcagatgagaaatgcctccttcaaggttttcttttgatttccttaacagtatgattcagcaagtttgctccctcaacagatattcattgagtgcccttaatatgacagacactctcttaattgcttgaaacacatcagtgaacaaagcagacaaaacctcggtttcatggagcttac

SEQ ID NO: 15430 - RNA, 1602 nt, Homo sapiens
  source 1..1602: mol_type = other RNA
gctgggattacaggcatgagccactgcgcctggcctctttgaatttttttaaaaacatcctggtgctaaaaggcagcaagattcataaatgcaaacaaacatataaataaacaaccaggccctcttcccttttaaataatctgtgaaataaaaataatctatctgcataggaaacaattatcaaatcagcatctacaatgtggcccaataaaagaaagggttttcatatttgatcctgtttttggttcctcaaaattaaaaacttggctccactctgtgctgtataatgatagattttttttaagaagagagagagtgggaattctcttgctgtttccatgggtttcatcatctttttttccatgactcataatggcttcttgcaaacactcttgttcccttgatctcatggagcgaatgaatgctcttaagctagttttcatcaaccagtcagcattcctcctgctttccaactgtgcatcctcagctggacacaaacattttccagtctactcattcacaaaataaacttctgagtattcttcaaagggctcggtccaacttgcccggggatattcgtgtatattgatctcactgatgcactgtggaagtaacttatagttctggaattgggggaagcacttcctggacttgatccaaaggcagcctctgcgtggtctctgctgaaagaacctgcacattcaatgctctcagtttctccgaatcacttcctcttaagagaacagatgtaggtttgtctctatgactctgccacttttgcactcttctctggccttcaagtattttgcggatagtgaggatgatcaaaaatataaaaactaatagaactaaaatataccaagtgatcttcatggaacaagtgatattttttatatccatctctaggtgcaaagaaatgtgtatacaatcattcgggtattccatgattctacaagtgtagtttatcgatttctccttgcttggctcatcctccatgattgttgatcttccagtgtggttttttagatgacaggtagtgttatattcctccaagtggtcaaccagaggagctacactgaagttaaagtgctgacaaggtgaatgaaaatcatttgctttcacttccattgatcctctcctgataagaacttttgatgtttgttcctgagaaataaaatccatgtttcctttagactcacaaaccaaacacgaggagcacattttaaattcacctgtgatgtcttggcaagtcctggtgaagttacgaaaattggagggatttagaaagattctcatgataatctgagtttcccttactggttgcagaaaagtcacaaaagaaaaatttaaggaggagagtgaataggtaaaattagattgcaaacacacttccagacatgatagctccaatgttctttctttcggtgtcttgaaatattccggcaaaattaaaatgaatgtgatcactattgccacaaataatttaaggagggctgtttttgtcatgtctcttcacatgacacaaatgtgttcccttgcagtacattcatggtatgttgcttcctgctttaagtttatctctgcagcactttaggttaatgc

SEQ ID NO: 15431 - RNA, 1660 nt, Homo sapiens
  source 1..1660: mol_type = other RNA
gctgggattacaggcatgagccactgcgcctggcctctttgaatttttttaaaaacatcctggtgctaaaaggcagcaagattcataaatgcaaacaaacatataaataaacaaccaggccctcttcccttttaaataatctgtgaaataaaaataatctatctgcataggaaacaattatcaaatcagcatctacaatgtggcccaataaaagaaagggttttcatatttgatcctgtttttggttcctcaaaattaaaaacttggctccactctgtgctgtataatgatagattttttttaagaagagagagagtgggaattctcttgctgtttccatgggtttcatcatctttttttccatgactcataatggcttcttgcaaacactcttgttcccttgatctcatggagcgaatgaatgctcttaagctagttttcatcaaccagtcagcattcctcctgctttccaactgtgcatcctcagctggacacaaacattttccagtctactcattcacaaaataaacttctgagtattcttcaaagggctcggtccaacttgcccggggatattcgtgtatattgatctcactgatgcactgtggaagtaacttatagttctggaattgggggaagcacttcctggacttgatccaaaggcagcctctgcgtggtctctgctgaaagaacctgcacattcaatgctctcagtttctccgaatcacttcctcttaagagaacagatgtaggtttgtctctatgactctgccacttttgcactcttctctggccttcaagtattttgcggatagtgaggatgatcaaaaatataaaaactaatagaactaaaatataccaagtgatcttcatggaacaagtgatattttttatatccatctctaggtgcaaagaaatgtgtatacaatcattcgggtattccatgattctacaagtgtagtttatcgatttctccttgcttggctcatcctccatgattgttgatcttccagtgtggttttttagatgacaggtagtgttatattcctccaagtggtcaaccagaggagctacactgaagttaaagtgctgacaaggtgaatgaaaatcatttgctttcacttccattgatcctctcctgataagaacttttgatgtttgttcctgagaaataaaatccatgtttcctttagactcacaaaccaaacacgaggagcacattttaaattcacctgtgatgtcttggcaagtcctggtgaagttacgaaaattggagggatttagaaagattctcatgataatctgagtttcccttactggttgcagaaaagtcacaaaagaaaaatttaaggaggagagtgaataggtaaaattagattgcaaacacacttccagacatgatagctccaatgttctttgtggaagcaatacttatgtttccattgcatcttgtttacatccctgtttcagttaattcctgtattttatttagttgtttgccagtcagttgtcctcccgactgaaaactccttgatcaaagagttgtctttcctttttgtagccccaggtttctttcggtgtcttgaaatattccggcaaaattaaaatgaatgtgatcactattgccacaaataatttaaggagggctgtttttgtcatg

SEQ ID NO: 15432 - RNA, 7561 nt, Homo sapiens
  source 1..7561: mol_type = other RNA
gctgggattacaggcatgagccactgcgcctggccttcaagcttcattttacaatcagtagacactgtcactaattattgagaaaatttatacaaatcaagggaaattcagagaaaagtcaaacagaagaaaaataatgagtctggaagaaaatatagcccagccattccttctctccaggcaggacctaagaagtgctctctgtggacacggcccaaaccagacaggccccttcctgcctgtgcccgatttccaagctggcccaaccaggctattccctcatagcctgtgtagtttacagtgttctacagattttttaaatcatattttaaacaagcttcactttcttcttctaagaatcatgagctgcaacattcctcattttctcagttgagtccctcagtaaagcccaaggtgtctgcaggcaggactgtcctaacctactagaactttccaccagagggctctgtctctgagacttccattttgatgcacatttttaaaaactggcacactttggtctgatacaagatcctgttccatgatgctttgattttatagacctcttggtcacagtctagttcatctggaaagttgtggaggggaaaataagatcacatgcattttacagaaggaaaatctaagaactaagacctagagagaagggtgaacagataacgtgttcatgaatcaggagattcatagcagagaaactgagaggagagacaagagtagggtgtcctgagtccaaaggctaccttcagaattcctgggctctggcttcatcccaggtttgctcttctggaagacctaacagatctaacctgcttctgatttttatttttgacaatatgcataggggcattaggacactagtaattttacttgagtgagcatattaggaagaggaagagggcaagttagagaataaagatgtttgggaatgagtcttcaacgcatccacagagtgaggagtggttttattttaggataaacgcagcctgttcagtgtcactttggaattcctccatcctttatgaccaagcctctttcctccttcctgcacgtctcttcttggggtgctgtctttcacctccttacaactggttaggtgcttcagctgacctcttagttggtctgcctaactctgaaagtcttctccctccaaagtgcctttacactaggaacagcctctgatgtatgcatcctgatattattttattttatttttattttttgagacatggtctcactctgttgcccagcctggagtgcagtggcaggatctcagctcactgcaacctccacctcccaggttcaagcaattctcccacctcagcctcccaagtagctgggattacaggtgtgcaccaccacgcccagctaatttttttgtattttaagtacagatggggttttgccatgctggccaggatcctctcaaattcctgacctcaagtgatccgcccaccttggcctcccaaagtgctgggattacaggcgtgagccaccgtgcccagctgcatcctgatatttaatgcttgccagaatttgattgcaccatgcttattggcttctatctttttttttttttcgagatggagtctcactctgtctctcccaggctggagtgcagtggtgtgatctcagctcactgcaacctccacttcctgggttcaagcgattctcctgtctcagcctccagagtagctgggactacagatgtgtgccaccacacctggctaatttcgtatttttagtagagatggggtttcaccatgttggccagactaatctcgaactcctgacctcaggtgatccgcctgccttggcctcccaaagtgttgggattacaggcgtgagccaccaccccagccggcttccgtttatctgtaattcccacatgtacaatgtagtgaggaaaacaaataattagttatgctgtaaggctgaatgagatgagttttagtgatagaaggaccaaagaggaaaaaacagcagtgtgaaaagatccctgattaattttgattcctgataccagggaaagctttacagaagaggtaccttttgaggtgggcattgaaggacatgtaaatggacatggggtgagggcacacatctggctgggacactctgccacacataggcaagggactgtgagcatgcatggtgcatctggagaggtgctctgaatacaccccactgatccaggcccctgctcatttttcatgcttctctcacttggaggccctctgtcttcctcattctctatccaaatttcatccatccttcaaggcccagcttcagccctgccccctcataaggtatttttctgactgttcatgctattacttgcagctgcagttcagcgttaactgtagtgtctgtgctggaattgtctcctgagctacacaagagcagacattatgcacatcttctactttggggccttgcagctcctaacatagtgctaatggtagttggtgctagatgagtctatggattcatttactgggactgatgtctttatctgcctaattgcagcccattgctgtccagcctaggactattcattgggatttaggagttagccgattatacttgctaacacataagggaaacacttccttaaatgatcatatgaatgtcttgctcagttgtgaatgattcttcctcattgaggagagttaatgcctgtgtaagctggctggtgatctgtttgtggggcatgccagggtggcggcactctgcctcagcttaaactctagttctctgagtctttggaactgggatgaacccagtttcatcatctgcaccatcatctcccaagttccttctggagaatgactctgcttcttgcaaggtcttctattttgatggttggattatacccagttccccagaagtgtgagaaatataagctggtcagttccttttggagagtgggaatactgggcatggctgcttcttctgctgaggctgcttggagtgatacagaaggaaatcttggccagaaagaaaatcctataaggcttctgaagtagcactccaagaaaagtgtcccagcagtctctagaccctgcagaaagaacattttccaacactccatttggagagtgtgtctacatggctgagagccacaactctgacagagacccacacagcactgtcatctgtgtttggacttactaagcctgttatgccctgcacaaagattcccagacaaagggatgagtgtgcttatatgcagcccacattctgctctccaagccatgcactcgggggaagggctgcatctgcctcaagcgaagggtacattttcctaatttgctcaagatgcgtggtgaaggccacgcaccagggatcttcacacatactgactgtgagcagagcatcttggctggtgtgccatggcctattacaggtgtgcaaaatattgatccccttctcccacagttactgggcagggttgttacctccagtcacaagaggcctctagtcatatgcagcttccagaagtgagcaatcttgcttgtttatcccagtgtgccataaaaatattattttctacatgtgctatgatgggaagaagtttgggaaaactatactaggtaacctgctttgtcattcattcagaagggagtcatttcaggaagggtatgcatccatttgtccatttaggcacaagctatgcccagcagaaggtttcctgctttgcttacaggctgagatgtggcagtttgcaatctcccagtaagagttgggcagagaagatctggatccagggaacctgccagtattggtggttgtaactcagtttccagagggagaattcagcccagcagcctagatcacaatttcatagcttgaagtcccaggaggtttactgtcctgtgtgctggctttccccatcttatcagcaaactgcacttcggaataaactgtgttcactggctcttccttggagggaagcacctcactccagtagctcctctgttgtgtggcccctctagggggcgccttgctcctagtcatggctcatctaacctggagccgggcccactgtgggacactcagtgcctcagcccatggaggctgccatggggtgacaatgggtcacgttcctgtcctcatagaaagatccgtggcatcacttccctgacatggtatttcctggttggaacctctggactcttggccgtggctgctttctagacaacaacaagcagaggcaatggctgcccatgactccctgtcatggagatggtggcacaggggtgtccatgaattgcatcagctcaccttggactgcaggatttcatcatagattctggactctgctggctgggtgttccttgaagccatgatatatgtgtatatggttttctttgaggcagcatctgtctcacaaataaatatagacccacagtctgtgaaaggtggtttttttagcaatgatctattccaatgttctctttttaagatgaagaaaggaagcccccagggattaaatggctgccatcctttgaaatggatgcttggatcctcagaatgtctcaggagtcacttggctgaggcctcacccacaggtcaatgggaattctcttctactctagagtccagattaggccaaagacaatttccccaacccctccctgtgtggccagtcaaatgtagctcttctacccaggatctcccttcatgtttctgacacttaccactgactgtcttgcatggctagttgactttccatgtcacggtcttagttttttaacttgattgattctttctagttatatactattttacattcttttggtgcagaccttgctgtaaccatctcaatgttaagcccatagtagatgtttcatgaacatttattgcttgtttgattgattcacagtctgtttttgtttgtttttgagacaagttctcactctgtcacccacgttggagtgcagtggtgcaccaactcatggctcactgcaacctctatcttctggactcaagtgatcctcccacctcagccttctgagtagctgggaccacaggtatgtgccaccacacccagcaaattttttgtatttttggtagagacagggtttcaccatgttgcccaggttggtcttgaactcctgagctcagctgatccacatgccttgatctcccaaagcgctgggattacaggcatgagccacagcaccctgccagttcacacagttaataaacatttattaagcaccttctatgtgccaggctctgtgtgaggccccagagaagaaaagacagtagacaagtctttccttttaagaatgtataggctagaagagacattcacgtcagtgtactcctttgctttggtactaacacagaacattttagggtcaaggtgaaaaaagaaggccagaattttgggccttcataatccagggcaccaacatacctacaaataacaggtctgagctgagcagtattacagggctccaacattcagagtttagtcctatcacttatttggtgagtatgagacaaactgagtgctctctcttgtctcatttatagatgcaaagaatagccctttctcttcccaagagtcagcgagggattgaagacaatatctctttgagggaccttgcagatcacctgtggttcaagcaggctatgccttctccccattgtgaggccatttgagtatggcacacgtcacaaatcccctcccccctagaatgcctcctccgtaccatgccccaggccaatcagttatcagtatactagctaacatttatcaagtacttactatgtactgggaattgggccaagtattttgtatttctaattccatttaatctacttaataagtatatacagcacaccttattactgtgaatattttacaactgagaaaatggaagcttacaatgataaaaaaactggtagctgataaatggtcaagctgggactttcacgcctagactgactgcaaatcacgtgcttagtcttaaccactctgttgggaactccccatccctcccaattgttattcaaggaactttgtggctgagaacttacaagggttcttagtgaaggtgttcaagcaggaacctgaggaatcagacccaaaggagagtcaggaacatggaagcagaagttccatgttttttattgtgattggtgggaaaaggaagttcttgggtggacatgggatgtgggtgaatcggagggtataatgattccttgagggtctaagatcaggttttctgaatggagaatggcacaactacagaatgatccagagggattcagagggacatagtgacaaccatggagtacaggattagtatatgtttctcaatgactctccaatagtcataatcaaaatacaatgaaattggaagtgaccctggagatcctctagtccaaacatttcacatgtgagggccctgagctggaaaggtgaacacactcgtacagtgaagcacagcttgttcatgtatgtactaagctcgaacccatgttctgggcccaccagctactggtgatctcaggaatggattctgaagaccattcagggtaatgtcataccatcctcagagccatcattctgggaggtggtggggtggagatcggaaaaaggcagattccctggaacaatgggcctttcagctaaaccttggataaatggcttcagtcccaggaggagagaaggtgagtttccacattttaccttctgggaaaatcctaccttgtcttctcttgaacaaacggaacaaaaacactgaagacagaatgagaacaagcagaaagaacatagccagcacgctcagcaacccggtgtggtgagtacggaagcccattgcgatgtctgcacagagctgccgggcagagatggagtcagaattgttgctgacagggttctgggctgtacacgtgtaagtcagctcttggtcctcaggagtctggaagatttgaaggacattaccctcttctcccaggggactccaattgtatgtcacattcttttcttctttctctacagagcatgtcagtgtgacattacaggtgctgttcacagatgccattaaactctgtgtaatttttggtttcccaagccgacgatagatttgcaggttgtagcgcttggtggtggtgtagggatcagcctgtgtatttatgtctgctttgtagtctcctgcgtcttccatcctcagatcgctaatgaccagattgtagttcggacctaaggcatgtatccgttcataataatttctgtgggtcacagtaactacgggtgctgtttctgagtctcctggtgttacataagcaacagatgttttagaagtccaagcaatgattttaacttgccgtggttcttggatatttacagggaaagtgactgactctcccagaatcccattcactgtgaagatttctgagtcttttccagctgcttccggccaggtttgcaggcaaaggagcaagatccataggtggtgctgagccatctctttcagggtctaaccttctgtggaaaagcacggcactgttctagcagagtcagttt

SEQ ID NO: 15433 - RNA, 4943 nt, Homo sapiens
  source 1..4943: mol_type = other RNA
gctgggattacaggcatgagccactgcgcctggccttcaagcttcattttacaatcagtagacactgtcactaattattgagaaaatttatacaaatcaagggaaattcagagaaaagtcaaacagaagaaaaataatgagtctggaagaaaatatagcccagccattccttctctccaggcaggacctaagaagtgctctctgtggacacggcccaaaccagacaggccccttcctgcctgtgcccgatttccaagctggcccaaccaggctattccctcatagcctgtgtagtttacagtgttctacagattttttaaatcatattttaaacaagcttcactttcttcttctaagaatcatgagctgcaacattcctcattttctcagttgagtccctcagtaaagcccaaggtgtctgcaggcaggactgtcctaacctactagaactttccaccagagggctctgtctctgagacttccattttgatgcacatttttaaaaactggcacactttggtctgatacaagatcctgttccatgatgctttgattttatagacctcttggtcacagtctagttcatctggaaagttgtggaggggaaaataagatcacatgcattttacagaaggaaaatctaagaactaagacctagagagaagggtgaacagataacgtgttcatgaatcaggagattcatagcagagaaactgagaggagagacaagagtagggtgtcctgagtccaaaggctaccttcagaattcctgggctctggcttcatcccaggtttgctcttctggaagacctaacagatctaacctgcttctgatttttatttttgacaatatgcataggggcattaggacactagtaattttacttgagtgagcatattaggaagaggaagagggcaagttagagaataaagatgtttgggaatgagtcttcaacgcatccacagagtgaggagtggttttattttaggataaacgcagcctgttcagtgtcactttggaattcctccatcctttatgaccaagcctctttcctccttcctgcacgtctcttcttggggtgctgtctttcacctccttacaactggttaggtgcttcagctgacctcttagttggtctgcctaactctgaaagtcttctccctccaaagtgcctttacactaggaacagcctctgatgtatgcatcctgatattattttattttatttttattttttgagacatggtctcactctgttgcccagcctggagtgcagtggcaggatctcagctcactgcaacctccacctcccaggttcaagcaattctcccacctcagcctcccaagtagctgggattacaggtgtgcaccaccacgcccagctaatttttttgtattttaagtacagatggggttttgccatgctggccaggatcctctcaaattcctgacctcaagtgatccgcccaccttggcctcccaaagtgctgggattacaggcgtgagccaccgtgcccagctgcatcctgatatttaatgcttgccagaatttgattgcaccatgcttattggcttctatctttttttttttttcgagatggagtctcactctgtctctcccaggctggagtgcagtggtgtgatctcagctcactgcaacctccacttcctgggttcaagcgattctcctgtctcagcctccagagtagctgggactacagatgtgtgccaccacacctggctaatttcgtatttttagtagagatggggtttcaccatgttggccagactaatctcgaactcctgacctcaggtgatccgcctgccttggcctcccaaagtgttgggattacaggcgtgagccaccaccccagccggcttccgtttatctgtaattcccacatgtacaatgtagtgaggaaaacaaataattagttatgctgtaaggctgaatgagatgagttttagtgatagaaggaccaaagaggaaaaaacagcagtgtgaaaagatccctgattaattttgattcctgataccagggaaagctttacagaagaggtaccttttgaggtgggcattgaaggacatgtaaatggacatggggtgagggcacacatctggctgggacactctgccacacataggcaagggactgtgagcatgcatggtgcatctggagaggtgctctgaatacaccccactgatccaggcccctgctcatttttcatgcttctctcacttggaggccctctgtcttcctcattctctatccaaatttcatccatccttcaaggcccagcttcagccctgccccctcataaggtatttttctgactgttcatgctattacttgcagctgcagttcagcgttaactgtagtgtctgtgctggaattgtctcctgagctacacaagagcagacattatgcacatcttctactttggggccttgcagctcctaacatagtgctaatggtagttggtgctagatgagtctatggattcatttactgggactgatgtctttatctgcctaattgcagcccattgctgtccagcctaggactattcattgggatttaggagttagccgattatacttgctaacacataagggaaacacttccttaaatgatcatatgaatgtcttgctcagttgtgaatgattcttcctcattgaggagagttaatgcctgtgtaagctggctggtgatctgtttgtggggcatgccagggtggcggcactctgcctcagcttaaactctagttctctgagtctttggaactgggatgaacccagtttcatcatctgcaccatcatctcccaagttccttctggagaatgactctgcttcttgcaaggtcttctattttgatggttggattatacccagttccccagaagtgtgagaaatataagctggtcagttccttttggagagtgggaatactgggcatggctgcttcttctgctgaggctgcttggagtgatacagaaggaaatcttggccagaaagaaaatcctataaggcttctgaagtagcactccaagaaaagtgtcccagcagtctctagaccctgcagaaagaacattttccaacactccatttggagagtgtgtctacatggctgagagccacaactctgacagagacccacacagcactgtcatctgtgtttggacttactaagcctgttatgccctgcacaaagattcccagacaaagggatgagtgtgcttatatgcagcccacattctgctctccaagccatgcactcgggggaagggctgcatctgcctcaagcgaagggtacattttcctaatttgctcaagatgcgtggtgaaggccacgcaccagggatcttcacacatactgactgtgagcagagcatcttggctggtgtgccatggcctattacaggtgtgcaaaatattgatccccttctcccacagttactgggcagggttgttacctccagtcacaagaggcctctagtcatatgcagcttccagaagtgagcaatcttgcttgtttatcccagtgtgccataaaaatattattttctacatgtgctatgatgggaagaagtttgggaaaactatactaggtaacctgctttgtcattcattcagaagggagtcatttcaggaagggtatgcatccatttgtccatttaggcacaagctatgcccagcagaaggtttcctgctttgcttacaggctgagatgtggcagtttgcaatctcccagtaagagttgggcagagaagatctggatccagggaacctgccagtattggtggttgtaactcagtttccagagggagaattcagcccagcagcctagatcacaatttcatagcttgaagtcccaggaggtttactgtcctgtgtgctggctttccccatcttatcagcaaactgcacttcggaataaactgtgttcactggctcttccttggagggaagcaccttggactgcaggatttcatcatagattctggactctgctggctgggtgttccttgaagccatgatatatgtgtatatggttttctttgaggcagcataagggttcttagtgaaggtgttcaagcaggaaccttctgggaaaatcctaccttgtcttctcttgaacaaacggaacaaaaacactgaagacagaatgagaacaagcagaaagaacatagccagcacgctcagcaacccggtgtggtgagtacggaagcccattgcgatgtctgcacagagctgccgggcagagatggagtcagaattgttgctgacagggttctgggctgtacacgtgtaagtcagctcttggtcctcaggagtctggaagatttgaaggacattaccctcttctcccaggggactccaattgtatgtcacattcttttcttctttctctacagagcatgtcagtgtgacattacaggtgctgttcacagatgccattaaactctgtgtaatttttggtttcccaagccgacgatagatttgcaggttgtagcgcttggtggtggtgtagggatcagcctgtgtatttatgtctgctttgtagtctcctgcgtcttccatcctcagatcgctaatgaccagattgtagttcggacctaaggcatgtatccgttcataataatttctgtgggtcacagtaactacgggtgctgtttctgagtctcctggtgttacataagcaacagatgttttagaagtccaagcaatgattttaacttgccgtggttcttggatatttacagggaaagtgactgactctcccagaatcccattcactgtgaagatttctgagtcttttccagctgcttccggccaggtttgcaggcaaaggagcaagatccataggtggtgctgagccatctctttcagggtctaaccttctgtggaaaagcacggcactgttctagcagagtcagttt

SEQ ID NO: 15434 - RNA, 4602 nt, Homo sapiens
  source 1..4602: mol_type = other RNA
gctgggattacaggcatgagccactgcgcctggccttcaagcttcattttacaatcagtagacactgtcactaattattgagaaaatttatacaaatcaagggaaattcagagaaaagtcaaacagaagaaaaataatgagtctggaagaaaatatagcccagccattccttctctccaggcaggacctaagaagtgctctctgtggacacggcccaaaccagacaggccccttcctgcctgtgcccgatttccaagctggcccaaccaggctattccctcatagcctgtgtagtttacagtgttctacagattttttaaatcatattttaaacaagcttcactttcttcttctaagaatcatgagctgcaacattcctcattttctcagttgagtccctcagtaaagcccaaggtgtctgcaggcaggactgtcctaacctactagaactttccaccagagggctctgtctctgagacttccattttgatgcacatttttaaaaactggcacactttggtctgatacaagatcctgttccatgatgctttgattttatagacctcttggtcacagtctagttcatctggaaagttgtggaggggaaaataagatcacatgcattttacagaaggaaaatctaagaactaagacctagagagaagggtgaacagataacgtgttcatgaatcaggagattcatagcagagaaactgagaggagagacaagagtagggtgtcctgagtccaaaggctaccttcagaattcctgggctctggcttcatcccaggtttgctcttctggaagacctaacagatctaacctgcttctgatttttatttttgacaatatgcataggggcattaggacactagtaattttacttgagtgagcatattaggaagaggaagagggcaagttagagaataaagatgtttgggaatgagtcttcaacgcatccacagagtgaggagtggttttattttaggataaacgcagcctgttcagtgtcactttggaattcctccatcctttatgaccaagcctctttcctccttcctgcacgtctcttcttggggtgctgtctttcacctccttacaactggttaggtgcttcagctgacctcttagttggtctgcctaactctgaaagtcttctccctccaaagtgcctttacactaggaacagcctctgatgtatgcatcctgatattattttattttatttttattttttgagacatggtctcactctgttgcccagcctggagtgcagtggcaggatctcagctcactgcaacctccacctcccaggttcaagcaattctcccacctcagcctcccaagtagctgggattacaggtgtgcaccaccacgcccagctaatttttttgtattttaagtacagatggggttttgccatgctggccaggatcctctcaaattcctgacctcaagtgatccgcccaccttggcctcccaaagtgctgggattacaggcgtgagccaccgtgcccagctgcatcctgatatttaatgcttgccagaatttgattgcaccatgcttattggcttctatctttttttttttttcgagatggagtctcactctgtctctcccaggctggagtgcagtggtgtgatctcagctcactgcaacctccacttcctgggttcaagcgattctcctgtctcagcctccagagtagctgggactacagatgtgtgccaccacacctggctaatttcgtatttttagtagagatggggtttcaccatgttggccagactaatctcgaactcctgacctcaggtgatccgcctgccttggcctcccaaagtgttgggattacaggcgtgagccaccaccccagccggcttccgtttatctgtaattcccacatgtacaatgtagtgaggaaaacaaataattagttatgctgtaaggctgaatgagatgagttttagtgatagaaggaccaaagaggaaaaaacagcagtgtgaaaagatccctgattaattttgattcctgataccagggaaagctttacagaagaggtaccttttgaggtgggcattgaaggacatgtaaatggacatggggtgagggcacacatctggctgggacactctgccacacataggcaagggactgtgagcatgcatggtgcatctggagaggtgctctgaatacaccccactgatccaggcccctgctcatttttcatgcttctctcacttggaggccctctgtcttcctcattctctatccaaatttcatccatccttcaaggcccagcttcagccctgccccctcataaggtatttttctgactgttcatgctattacttgcagctgcagttcagcgttaactgtagtgtctgtgctggaattgtctcctgagctacacaagagcagacattatgcacatcttctactttggggccttgcagctcctaacatagtgctaatggtagttggtgctagatgagtctatggattcatttactgggactgatgtctttatctgcctaattgcagcccattgctgtccagcctaggactattcattgggatttaggagttagccgattatacttgctaacacataagggaaacacttccttaaatgatcatatgaatgtcttgctcagttgtgaatgattcttcctcattgaggagagttaatgcctgtgtaagctggctggtgatctgtttgtggggcatgccagggtggcggcactctgcctcagcttaaactctagttctctgagtctttggaactgggatgaacccagtttcatcatctgcaccatcatctcccaagttccttctggagaatgactctgcttcttgcaaggtcttctattttgatggttggattatacccagttccccagaagtgtgagaaatataagctggtcagttccttttggagagtgggaatactgggcatggctgcttcttctgctgaggctgcttggagtgatacagaaggaaatcttggccagaaagaaaatcctataaggcttctgaagtagcactccaagaaaagtgtcccagcagtctctagaccctgcagaaagaacattttccaacactccatttggagagtgtgtctacatggctgagagccacaactctgacagagacccacacagcactgtcatctgtgtttggacttactaagcctgttatgccctgcacaaagattcccagacaaagggatgagtgtgcttatatgcagcccacattctgctctccaagccatgcactcgggggaagggctgcatctgcctcaagcgaagggtacattttcctaatttgctcaagatgcgtggtgaaggccacgcaccagggatcttcacacatactgactgtgagcagagcatcttggctggtgtgccatggcctattacaggtgtgcaaaatattgatccccttctcccacagttactgggcagggttgttacctccagtcacaagaggcctctagtcatatgcagcttccagaagtgagcaatcttgcttgtttatcccagtgtgccataaaaatattattttctacatgtgctatgatgggaagaagtttgggaaaactatactaggtaacctgctttgtcattcattcagaagggagtcatttcaggaagggtatgcatccatttgtccatttaggcacaagctatgcccagcagaaggtttcctgctttgcttacaggctgagatgtggcagtttgcaatctcccagtaagagttgggcagagaagatctggatccagggaacctgccagtattggtggttgtaactcagtttccagagggagaattcagcccagcagcctagatcacaatttcatagcttgaagtcccaggaggtttactgtcctgtgtgctggctttccccatcttatcagcaaactgcacttcggaataaactgtgttcactggctcttccttggagggaagcaccttggactgcaggatttcatcatagattctggactctgctggctgggtgttccttgaagccatgatatatgtgtatatggttttctttgaggcagcataagggttcttagtgaaggtgttcaagcaggaaccttgtcttctcttgaacaaacggaacaaaaacactgaagacagaatgagaacaagcagaaagaacatagccagcacgctcagcaacccggtgtggtgagtacggaagcccattgcgatgtctgcacagagctgccgggcagagatggagtcagaattgttgctgacagggttctgggctgtacacgtgtaagtcagctcttggtcctcaggagtctggaagatttgaaggacattaccctcttctcccaggggactccaattgtatgtcacattcttttcttctttctctacagagcatgtcagtgtgacattacaggtgctgttcacagatgccattaaactctgtgtaatttttggtttcccaagccgacaggtttgcaggcaaaggagcaagatccataggtggtgctgagccatctctttcagggtctaaccttctgtggaaaagcacggcactgttctagcagagtcagtttcacttgagttttcttcctc

SEQ ID NO: 15435 - RNA, 4925 nt, Homo sapiens
  source 1..4925: mol_type = other RNA
gctgggattacaggcatgagccactgcgcctggccttcaagcttcattttacaatcagtagacactgtcactaattattgagaaaatttatacaaatcaagggaaattcagagaaaagtcaaacagaagaaaaataatgagtctggaagaaaatatagcccagccattccttctctccaggcaggacctaagaagtgctctctgtggacacggcccaaaccagacaggccccttcctgcctgtgcccgatttccaagctggcccaaccaggctattccctcatagcctgtgtagtttacagtgttctacagattttttaaatcatattttaaacaagcttcactttcttcttctaagaatcatgagctgcaacattcctcattttctcagttgagtccctcagtaaagcccaaggtgtctgcaggcaggactgtcctaacctactagaactttccaccagagggctctgtctctgagacttccattttgatgcacatttttaaaaactggcacactttggtctgatacaagatcctgttccatgatgctttgattttatagacctcttggtcacagtctagttcatctggaaagttgtggaggggaaaataagatcacatgcattttacagaaggaaaatctaagaactaagacctagagagaagggtgaacagataacgtgttcatgaatcaggagattcatagcagagaaactgagaggagagacaagagtagggtgtcctgagtccaaaggctaccttcagaattcctgggctctggcttcatcccaggtttgctcttctggaagacctaacagatctaacctgcttctgatttttatttttgacaatatgcataggggcattaggacactagtaattttacttgagtgagcatattaggaagaggaagagggcaagttagagaataaagatgtttgggaatgagtcttcaacgcatccacagagtgaggagtggttttattttaggataaacgcagcctgttcagtgtcactttggaattcctccatcctttatgaccaagcctctttcctccttcctgcacgtctcttcttggggtgctgtctttcacctccttacaactggttaggtgcttcagctgacctcttagttggtctgcctaactctgaaagtcttctccctccaaagtgcctttacactaggaacagcctctgatgtatgcatcctgatattattttattttatttttattttttgagacatggtctcactctgttgcccagcctggagtgcagtggcaggatctcagctcactgcaacctccacctcccaggttcaagcaattctcccacctcagcctcccaagtagctgggattacaggtgtgcaccaccacgcccagctaatttttttgtattttaagtacagatggggttttgccatgctggccaggatcctctcaaattcctgacctcaagtgatccgcccaccttggcctcccaaagtgctgggattacaggcgtgagccaccgtgcccagctgcatcctgatatttaatgcttgccagaatttgattgcaccatgcttattggcttctatctttttttttttttcgagatggagtctcactctgtctctcccaggctggagtgcagtggtgtgatctcagctcactgcaacctccacttcctgggttcaagcgattctcctgtctcagcctccagagtagctgggactacagatgtgtgccaccacacctggctaatttcgtatttttagtagagatggggtttcaccatgttggccagactaatctcgaactcctgacctcaggtgatccgcctgccttggcctcccaaagtgttgggattacaggcgtgagccaccaccccagccggcttccgtttatctgtaattcccacatgtacaatgtagtgaggaaaacaaataattagttatgctgtaaggctgaatgagatgagttttagtgatagaaggaccaaagaggaaaaaacagcagtgtgaaaagatccctgattaattttgattcctgataccagggaaagctttacagaagaggtaccttttgaggtgggcattgaaggacatgtaaatggacatggggtgagggcacacatctggctgggacactctgccacacataggcaagggactgtgagcatgcatggtgcatctggagaggtgctctgaatacaccccactgatccaggcccctgctcatttttcatgcttctctcacttggaggccctctgtcttcctcattctctatccaaatttcatccatccttcaaggcccagcttcagccctgccccctcataaggtatttttctgactgttcatgctattacttgcagctgcagttcagcgttaactgtagtgtctgtgctggaattgtctcctgagctacacaagagcagacattatgcacatcttctactttggggccttgcagctcctaacatagtgctaatggtagttggtgctagatgagtctatggattcatttactgggactgatgtctttatctgcctaattgcagcccattgctgtccagcctaggactattcattgggatttaggagttagccgattatacttgctaacacataagggaaacacttccttaaatgatcatatgaatgtcttgctcagttgtgaatgattcttcctcattgaggagagttaatgcctgtgtaagctggctggtgatctgtttgtggggcatgccagggtggcggcactctgcctcagcttaaactctagttctctgagtctttggaactgggatgaacccagtttcatcatctgcaccatcatctcccaagttccttctggagaatgactctgcttcttgcaaggtcttctattttgatggttggattatacccagttccccagaagtgtgagaaatataagctggtcagttccttttggagagtgggaatactgggcatggctgcttcttctgctgaggctgcttggagtgatacagaaggaaatcttggccagaaagaaaatcctataaggcttctgaagtagcactccaagaaaagtgtcccagcagtctctagaccctgcagaaagaacattttccaacactccatttggagagtgtgtctacatggctgagagccacaactctgacagagacccacacagcactgtcatctgtgtttggacttactaagcctgttatgccctgcacaaagattcccagacaaagggatgagtgtgcttatatgcagcccacattctgctctccaagccatgcactcgggggaagggctgcatctgcctcaagcgaagggtacattttcctaatttgctcaagatgcgtggtgaaggccacgcaccagggatcttcacacatactgactgtgagcagagcatcttggctggtgtgccatggcctattacaggtgtgcaaaatattgatccccttctcccacagttactgggcagggttgttacctccagtcacaagaggcctctagtcatatgcagcttccagaagtgagcaatcttgcttgtttatcccagtgtgccataaaaatattattttctacatgtgctatgatgggaagaagtttgggaaaactatactaggtaacctgctttgtcattcattcagaagggagtcatttcaggaagggtatgcatccatttgtccatttaggcacaagctatgcccagcagaaggtttcctgctttgcttacaggctgagatgtggcagtttgcaatctcccagtaagagttgggcagagaagatctggatccagggaacctgccagtattggtggttgtaactcagtttccagagggagaattcagcccagcagcctagatcacaatttcatagcttgaagtcccaggaggtttactgtcctgtgtgctggctttccccatcttatcagcaaactgcacttcggaataaactgtgttcactggctcttccttggagggaagcaccttggactgcaggatttcatcatagattctggactctgctggctgggtgttccttgaagccatgatatatgtgtatatggttttctttgaggcagcataagggttcttagtgaaggtgttcaagcaggaaccttgtcttctcttgaacaaacggaacaaaaacactgaagacagaatgagaacaagcagaaagaacatagccagcacgctcagcaacccggtgtggtgagtacggaagcccattgcgatgtctgcacagagctgccgggcagagatggagtcagaattgttgctgacagggttctgggctgtacacgtgtaagtcagctcttggtcctcaggagtctggaagatttgaaggacattaccctcttctcccaggggactccaattgtatgtcacattcttttcttctttctctacagagcatgtcagtgtgacattacaggtgctgttcacagatgccattaaactctgtgtaatttttggtttcccaagccgacgatagatttgcaggttgtagcgcttggtggtggtgtagggatcagcctgtgtatttatgtctgctttgtagtctcctgcgtcttccatcctcagatcgctaatgaccagattgtagttcggacctaaggcatgtatccgttcataataatttctgtgggtcacagtaactacgggtgctgtttctgagtctcctggtgttacataagcaacagatgttttagaagtccaagcaatgattttaacttgccgtggttcttggatatttacagggaaagtgactgactctcccagaatcccattcactgtgaagatttctgagtcttttccagctgcttccggccaggtttgcaggcaaaggagcaagatccataggtggtgctgagccatctctttcagggtctaaccttctgtggaaaagcacggcactgttctagcagagtcagttt

SEQ ID NO: 15436 - RNA, 4550 nt, Homo sapiens
  source 1..4550: mol_type = other RNA
gctgggattacaggcatgagccactgcgcctggccttcaagcttcattttacaatcagtagacactgtcactaattattgagaaaatttatacaaatcaagggaaattcagagaaaagtcaaacagaagaaaaataatgagtctggaagaaaatatagcccagccattccttctctccaggcaggacctaagaagtgctctctgtggacacggcccaaaccagacaggccccttcctgcctgtgcccgatttccaagctggcccaaccaggctattccctcatagcctgtgtagtttacagtgttctacagattttttaaatcatattttaaacaagcttcactttcttcttctaagaatcatgagctgcaacattcctcattttctcagttgagtccctcagtaaagcccaaggtgtctgcaggcaggactgtcctaacctactagaactttccaccagagggctctgtctctgagacttccattttgatgcacatttttaaaaactggcacactttggtctgatacaagatcctgttccatgatgctttgattttatagacctcttggtcacagtctagttcatctggaaagttgtggaggggaaaataagatcacatgcattttacagaaggaaaatctaagaactaagacctagagagaagggtgaacagataacgtgttcatgaatcaggagattcatagcagagaaactgagaggagagacaagagtagggtgtcctgagtccaaaggctaccttcagaattcctgggctctggcttcatcccaggtttgctcttctggaagacctaacagatctaacctgcttctgatttttatttttgacaatatgcataggggcattaggacactagtaattttacttgagtgagcatattaggaagaggaagagggcaagttagagaataaagatgtttgggaatgagtcttcaacgcatccacagagtgaggagtggttttattttaggataaacgcagcctgttcagtgtcactttggaattcctccatcctttatgaccaagcctctttcctccttcctgcacgtctcttcttggggtgctgtctttcacctccttacaactggttaggtgcttcagctgacctcttagttggtctgcctaactctgaaagtcttctccctccaaagtgcctttacactaggaacagcctctgatgtatgcatcctgatattattttattttatttttattttttgagacatggtctcactctgttgcccagcctggagtgcagtggcaggatctcagctcactgcaacctccacctcccaggttcaagcaattctcccacctcagcctcccaagtagctgggattacaggtgtgcaccaccacgcccagctaatttttttgtattttaagtacagatggggttttgccatgctggccaggatcctctcaaattcctgacctcaagtgatccgcccaccttggcctcccaaagtgctgggattacaggcgtgagccaccgtgcccagctgcatcctgatatttaatgcttgccagaatttgattgcaccatgcttattggcttctatctttttttttttttcgagatggagtctcactctgtctctcccaggctggagtgcagtggtgtgatctcagctcactgcaacctccacttcctgggttcaagcgattctcctgtctcagcctccagagtagctgggactacagatgtgtgccaccacacctggctaatttcgtatttttagtagagatggggtttcaccatgttggccagactaatctcgaactcctgacctcaggtgatccgcctgccttggcctcccaaagtgttgggattacaggcgtgagccaccaccccagccggcttccgtttatctgtaattcccacatgtacaatgtagtgaggaaaacaaataattagttatgctgtaaggctgaatgagatgagttttagtgatagaaggaccaaagaggaaaaaacagcagtgtgaaaagatccctgattaattttgattcctgataccagggaaagctttacagaagaggtaccttttgaggtgggcattgaaggacatgtaaatggacatggggtgagggcacacatctggctgggacactctgccacacataggcaagggactgtgagcatgcatggtgcatctggagaggtgctctgaatacaccccactgatccaggcccctgctcatttttcatgcttctctcacttggaggccctctgtcttcctcattctctatccaaatttcatccatccttcaaggcccagcttcagccctgccccctcataaggtatttttctgactgttcatgctattacttgcagctgcagttcagcgttaactgtagtgtctgtgctggaattgtctcctgagctacacaagagcagacattatgcacatcttctactttggggccttgcagctcctaacatagtgctaatggtagttggtgctagatgagtctatggattcatttactgggactgatgtctttatctgcctaattgcagcccattgctgtccagcctaggactattcattgggatttaggagttagccgattatacttgctaacacataagggaaacacttccttaaatgatcatatgaatgtcttgctcagttgtgaatgattcttcctcattgaggagagttaatgcctgtgtaagctggctggtgatctgtttgtggggcatgccagggtggcggcactctgcctcagcttaaactctagttctctgagtctttggaactgggatgaacccagtttcatcatctgcaccatcatctcccaagttccttctggagaatgactctgcttcttgcaaggtcttctattttgatggttggattatacccagttccccagaagtgtgagaaatataagctggtcagttccttttggagagtgggaatactgggcatggctgcttcttctgctgaggctgcttggagtgatacagaaggaaatcttggccagaaagaaaatcctataaggcttctgaagtagcactccaagaaaagtgtcccagcagtctctagaccctgcagaaagaacattttccaacactccatttggagagtgtgtctacatggctgagagccacaactctgacagagacccacacagcactgtcatctgtgtttggacttactaagcctgttatgccctgcacaaagattcccagacaaagggatgagtgtgcttatatgcagcccacattctgctctccaagccatgcactcgggggaagggctgcatctgcctcaagcgaagggtacattttcctaatttgctcaagatgcgtggtgaaggccacgcaccagggatcttcacacatactgactgtgagcagagcatcttggctggtgtgccatggcctattacaggtgtgcaaaatattgatccccttctcccacagttactgggcagggttgttacctccagtcacaagaggcctctagtcatatgcagcttccagaagtgagcaatcttgcttgtttatcccagtgtgccataaaaatattattttctacatgtgctatgatgggaagaagtttgggaaaactatactaggtaacctgctttgtcattcattcagaagggagtcatttcaggaagggtatgcatccatttgtccatttaggcacaagctatgcccagcagaaggtttcctgctttgcttacaggctgagatgtggcagtttgcaatctcccagtaagagttgggcagagaagatctggatccagggaacctgccagtattggtggttgtaactcagtttccagagggagaattcagcccagcagcctagatcacaatttcatagcttgaagtcccaggaggtttactgtcctgtgtgctggctttccccatcttatcagcaaactgcacttcggaataaactgtgttcactggctcttccttggagggaagcaccttggactgcaggatttcatcatagattctggactctgctggctgggtgttccttgaagccatgatatatgtgtatatggttttctttgaggcagcatcttgtcttctcttgaacaaacggaacaaaaacactgaagacagaatgagaacaagcagaaagaacatagccagcacgctcagcaacccggtgtggtgagtacggaagcccattgcgatgtctgcacagagctgccgggcagagatggagtcagaattgttgctgacagggttctgggctgtacacgtgtaagtcagctcttggtcctcaggagtctggaagatttgaaggacattaccctcttctcccaggggactccaattgtatgtcacattcttttcttctttctctacagagcatgtcagtgtgacattacaggtgctgttcacagatgccattaaactctgtgtaatttttggtttcccaagccgacaggtttgcaggcaaaggagcaagatccataggtggtgctgagccatctctttcagggtctaaccttctgtggaaaagcacggcactgttctagcagagtcagttt

SEQ ID NO: 15437 - RNA, 4892 nt, Homo sapiens
  source 1..4892: mol_type = other RNA
gctgggattacaggcatgagccactgcgcctggccttcaagcttcattttacaatcagtagacactgtcactaattattgagaaaatttatacaaatcaagggaaattcagagaaaagtcaaacagaagaaaaataatgagtctggaagaaaatatagcccagccattccttctctccaggcaggacctaagaagtgctctctgtggacacggcccaaaccagacaggccccttcctgcctgtgcccgatttccaagctggcccaaccaggctattccctcatagcctgtgtagtttacagtgttctacagattttttaaatcatattttaaacaagcttcactttcttcttctaagaatcatgagctgcaacattcctcattttctcagttgagtccctcagtaaagcccaaggtgtctgcaggcaggactgtcctaacctactagaactttccaccagagggctctgtctctgagacttccattttgatgcacatttttaaaaactggcacactttggtctgatacaagatcctgttccatgatgctttgattttatagacctcttggtcacagtctagttcatctggaaagttgtggaggggaaaataagatcacatgcattttacagaaggaaaatctaagaactaagacctagagagaagggtgaacagataacgtgttcatgaatcaggagattcatagcagagaaactgagaggagagacaagagtagggtgtcctgagtccaaaggctaccttcagaattcctgggctctggcttcatcccaggtttgctcttctggaagacctaacagatctaacctgcttctgatttttatttttgacaatatgcataggggcattaggacactagtaattttacttgagtgagcatattaggaagaggaagagggcaagttagagaataaagatgtttgggaatgagtcttcaacgcatccacagagtgaggagtggttttattttaggataaacgcagcctgttcagtgtcactttggaattcctccatcctttatgaccaagcctctttcctccttcctgcacgtctcttcttggggtgctgtctttcacctccttacaactggttaggtgcttcagctgacctcttagttggtctgcctaactctgaaagtcttctccctccaaagtgcctttacactaggaacagcctctgatgtatgcatcctgatattattttattttatttttattttttgagacatggtctcactctgttgcccagcctggagtgcagtggcaggatctcagctcactgcaacctccacctcccaggttcaagcaattctcccacctcagcctcccaagtagctgggattacaggtgtgcaccaccacgcccagctaatttttttgtattttaagtacagatggggttttgccatgctggccaggatcctctcaaattcctgacctcaagtgatccgcccaccttggcctcccaaagtgctgggattacaggcgtgagccaccgtgcccagctgcatcctgatatttaatgcttgccagaatttgattgcaccatgcttattggcttctatctttttttttttttcgagatggagtctcactctgtctctcccaggctggagtgcagtggtgtgatctcagctcactgcaacctccacttcctgggttcaagcgattctcctgtctcagcctccagagtagctgggactacagatgtgtgccaccacacctggctaatttcgtatttttagtagagatggggtttcaccatgttggccagactaatctcgaactcctgacctcaggtgatccgcctgccttggcctcccaaagtgttgggattacaggcgtgagccaccaccccagccggcttccgtttatctgtaattcccacatgtacaatgtagtgaggaaaacaaataattagttatgctgtaaggctgaatgagatgagttttagtgatagaaggaccaaagaggaaaaaacagcagtgtgaaaagatccctgattaattttgattcctgataccagggaaagctttacagaagaggtaccttttgaggtgggcattgaaggacatgtaaatggacatggggtgagggcacacatctggctgggacactctgccacacataggcaagggactgtgagcatgcatggtgcatctggagaggtgctctgaatacaccccactgatccaggcccctgctcatttttcatgcttctctcacttggaggccctctgtcttcctcattctctatccaaatttcatccatccttcaaggcccagcttcagccctgccccctcataaggtatttttctgactgttcatgctattacttgcagctgcagttcagcgttaactgtagtgtctgtgctggaattgtctcctgagctacacaagagcagacattatgcacatcttctactttggggccttgcagctcctaacatagtgctaatggtagttggtgctagatgagtctatggattcatttactgggactgatgtctttatctgcctaattgcagcccattgctgtccagcctaggactattcattgggatttaggagttagccgattatacttgctaacacataagggaaacacttccttaaatgatcatatgaatgtcttgctcagttgtgaatgattcttcctcattgaggagagttaatgcctgtgtaagctggctggtgatctgtttgtggggcatgccagggtggcggcactctgcctcagcttaaactctagttctctgagtctttggaactgggatgaacccagtttcatcatctgcaccatcatctcccaagttccttctggagaatgactctgcttcttgcaaggtcttctattttgatggttggattatacccagttccccagaagtgtgagaaatataagctggtcagttccttttggagagtgggaatactgggcatggctgcttcttctgctgaggctgcttggagtgatacagaaggaaatcttggccagaaagaaaatcctataaggcttctgaagtagcactccaagaaaagtgtcccagcagtctctagaccctgcagaaagaacattttccaacactccatttggagagtgtgtctacatggctgagagccacaactctgacagagacccacacagcactgtcatctgtgtttggacttactaagcctgttatgccctgcacaaagattcccagacaaagggatgagtgtgcttatatgcagcccacattctgctctccaagccatgcactcgggggaagggctgcatctgcctcaagcgaagggtacattttcctaatttgctcaagatgcgtggtgaaggccacgcaccagggatcttcacacatactgactgtgagcagagcatcttggctggtgtgccatggcctattacaggtgtgcaaaatattgatccccttctcccacagttactgggcagggttgttacctccagtcacaagaggcctctagtcatatgcagcttccagaagtgagcaatcttgcttgtttatcccagtgtgccataaaaatattattttctacatgtgctatgatgggaagaagtttgggaaaactatactaggtaacctgctttgtcattcattcagaagggagtcatttcaggaagggtatgcatccatttgtccatttaggcacaagctatgcccagcagaaggtttcctgctttgcttacaggctgagatgtggcagtttgcaatctcccagtaagagttgggcagagaagatctggatccagggaacctgccagtattggtggttgtaactcagtttccagagggagaattcagcccagcagcctagatcacaatttcatagcttgaagtcccaggaggtttactgtcctgtgtgctggctttccccatcttatcagcaaactgcacttcggaataaactgtgttcactggctcttccttggagggaagcaccttggactgcaggatttcatcatagattctggactctgctggctgggtgttccttgaagccatgatatatgtgtatatggttttctttgaggcagcatcttgtcttctcttgaacaaacggaacaaaaacactgaagacagaatgagaacaagcagaaagaacatagccagcacgctcagcaacccggtgtggtgagtacggaagcccattgcgatgtctgcacagagctgccgggcagagatggagtcagaattgttgctgacagggttctgggctgtacacgtgtaagtcagctcttggtcctcaggagtctggaagatttgaaggacattaccctcttctcccaggggactccaattgtatgtcacattcttttcttctttctctacagagcatgtcagtgtgacattacaggtgctgttcacagatgccattaaactctgtgtaatttttggtttcccaagccgacgatagatttgcaggttgtagcgcttggtggtggtgtagggatcagcctgtgtatttatgtctgctttgtagtctcctgcgtcttccatcctcagatcgctaatgaccagattgtagttcggacctaaggcatgtatccgttcataataatttctgtgggtcacagtaactacgggtgctgtttctgagtctcctggtgttacataagcaacagatgttttagaagtccaagcaatgattttaacttgccgtggttcttggatatttacagggaaagtgactgactctcccagaatcccattcactgtgaagatttctgagtcttttccagctgcttccggccaggtttgcaggcaaaggagcaagatccataggtggtgctgagccatctctttcagggtctaaccttctgtggaaaagcacggcactgttctagcagagtcagttt

SEQ ID NO: 15438 - RNA, 4794 nt, Homo sapiens
  source 1..4794: mol_type = other RNA
gctgggattacaggcatgagccactgcgcctggccttcaagcttcattttacaatcagtagacactgtcactaattattgagaaaatttatacaaatcaagggaaattcagagaaaagtcaaacagaagaaaaataatgagtctggaagaaaatatagcccagccattccttctctccaggcaggacctaagaagtgctctctgtggacacggcccaaaccagacaggccccttcctgcctgtgcccgatttccaagctggcccaaccaggctattccctcatagcctgtgtagtttacagtgttctacagattttttaaatcatattttaaacaagcttcactttcttcttctaagaatcatgagctgcaacattcctcattttctcagttgagtccctcagtaaagcccaaggtgtctgcaggcaggactgtcctaacctactagaactttccaccagagggctctgtctctgagacttccattttgatgcacatttttaaaaactggcacactttggtctgatacaagatcctgttccatgatgctttgattttatagacctcttggtcacagtctagttcatctggaaagttgtggaggggaaaataagatcacatgcattttacagaaggaaaatctaagaactaagacctagagagaagggtgaacagataacgtgttcatgaatcaggagattcatagcagagaaactgagaggagagacaagagtagggtgtcctgagtccaaaggctaccttcagaattcctgggctctggcttcatcccaggtttgctcttctggaagacctaacagatctaacctgcttctgatttttatttttgacaatatgcataggggcattaggacactagtaattttacttgagtgagcatattaggaagaggaagagggcaagttagagaataaagatgtttgggaatgagtcttcaacgcatccacagagtgaggagtggttttattttaggataaacgcagcctgttcagtgtcactttggaattcctccatcctttatgaccaagcctctttcctccttcctgcacgtctcttcttggggtgctgtctttcacctccttacaactggttaggtgcttcagctgacctcttagttggtctgcctaactctgaaagtcttctccctccaaagtgcctttacactaggaacagcctctgatgtatgcatcctgatattattttattttatttttattttttgagacatggtctcactctgttgcccagcctggagtgcagtggcaggatctcagctcactgcaacctccacctcccaggttcaagcaattctcccacctcagcctcccaagtagctgggattacaggtgtgcaccaccacgcccagctaatttttttgtattttaagtacagatggggttttgccatgctggccaggatcctctcaaattcctgacctcaagtgatccgcccaccttggcctcccaaagtgctgggattacaggcgtgagccaccgtgcccagctgcatcctgatatttaatgcttgccagaatttgattgcaccatgcttattggcttctatctttttttttttttcgagatggagtctcactctgtctctcccaggctggagtgcagtggtgtgatctcagctcactgcaacctccacttcctgggttcaagcgattctcctgtctcagcctccagagtagctgggactacagatgtgtgccaccacacctggctaatttcgtatttttagtagagatggggtttcaccatgttggccagactaatctcgaactcctgacctcaggtgatccgcctgccttggcctcccaaagtgttgggattacaggcgtgagccaccaccccagccggcttccgtttatctgtaattcccacatgtacaatgtagtgaggaaaacaaataattagttatgctgtaaggctgaatgagatgagttttagtgatagaaggaccaaagaggaaaaaacagcagtgtgaaaagatccctgattaattttgattcctgataccagggaaagctttacagaagaggtaccttttgaggtgggcattgaaggacatgtaaatggacatggggtgagggcacacatctggctgggacactctgccacacataggcaagggactgtgagcatgcatggtgcatctggagaggtgctctgaatacaccccactgatccaggcccctgctcatttttcatgcttctctcacttggaggccctctgtcttcctcattctctatccaaatttcatccatccttcaaggcccagcttcagccctgccccctcataaggtatttttctgactgttcatgctattacttgcagctgcagttcagcgttaactgtagtgtctgtgctggaattgtctcctgagctacacaagagcagacattatgcacatcttctactttggggccttgcagctcctaacatagtgctaatggtagttggtgctagatgagtctatggattcatttactgggactgatgtctttatctgcctaattgcagcccattgctgtccagcctaggactattcattgggatttaggagttagccgattatacttgctaacacataagggaaacacttccttaaatgatcatatgaatgtcttgctcagttgtgaatgattcttcctcattgaggagagttaatgcctgtgtaagctggctggtgatctgtttgtggggcatgccagggtggcggcactctgcctcagcttaaactctagttctctgagtctttggaactgggatgaacccagtttcatcatctgcaccatcatctcccaagttccttctggagaatgactctgcttcttgcaaggtcttctattttgatggttggattatacccagttccccagaagtgtgagaaatataagctggtcagttccttttggagagtgggaatactgggcatggctgcttcttctgctgaggctgcttggagtgatacagaaggaaatcttggccagaaagaaaatcctataaggcttctgaagtagcactccaagaaaagtgtcccagcagtctctagaccctgcagaaagaacattttccaacactccatttggagagtgtgtctacatggctgagagccacaactctgacagagacccacacagcactgtcatctgtgtttggacttactaagcctgttatgccctgcacaaagattcccagacaaagggatgagtgtgcttatatgcagcccacattctgctctccaagccatgcactcgggggaagggctgcatctgcctcaagcgaagggtacattttcctaatttgctcaagatgcgtggtgaaggccacgcaccagggatcttcacacatactgactgtgagcagagcatcttggctggtgtgccatggcctattacaggtgtgcaaaatattgatccccttctcccacagttactgggcagggttgttacctccagtcacaagaggcctctagtcatatgcagcttccagaagtgagcaatcttgcttgtttatcccagtgtgccataaaaatattattttctacatgtgctatgatgggaagaagtttgggaaaactatactaggtaacctgctttgtcattcattcagaagggagtcatttcaggaagggtatgcatccatttgtccatttaggcacaagctatgcccagcagaaggtttcctgctttgcttacaggctgagatgtggcagtttgcaatctcccagtaagagttgggcagagaagatctggatccagggaacctgccagtattggtggttgtaactcagtttccagagggagaattcagcccagcagcctagatcacaatttcatagcttgaagtcccaggaggtttactgtcctgtgtgctggctttccccatcttatcagcaaactgcacttcggaataaactgtgttcactggctcttccttggagggaagcaccttgtcttctcttgaacaaacggaacaaaaacactgaagacagaatgagaacaagcagaaagaacatagccagcacgctcagcaacccggtgtggtgagtacggaagcccattgcgatgtctgcacagagctgccgggcagagatggagtcagaattgttgctgacagggttctgggctgtacacgtgtaagtcagctcttggtcctcaggagtctggaagatttgaaggacattaccctcttctcccaggggactccaattgtatgtcacattcttttcttctttctctacagagcatgtcagtgtgacattacaggtgctgttcacagatgccattaaactctgtgtaatttttggtttcccaagccgacgatagatttgcaggttgtagcgcttggtggtggtgtagggatcagcctgtgtatttatgtctgctttgtagtctcctgcgtcttccatcctcagatcgctaatgaccagattgtagttcggacctaaggcatgtatccgttcataataatttctgtgggtcacagtaactacgggtgctgtttctgagtctcctggtgttacataagcaacagatgttttagaagtccaagcaatgattttaacttgccgtggttcttggatatttacagggaaagtgactgactctcccagaatcccattcactgtgaagatttctgagtcttttccagctgcttccggccaggtttgcaggcaaaggagcaagatccataggtggtgctgagccatctctttcagggtctaaccttctgtggaaaagcacggcactgttctagcagagtcagttt

SEQ ID NO: 15439 - RNA, 9682 nt, Homo sapiens
  source 1..9682: mol_type = other RNA
gctgggattacaggcatgagccactgcgcctggccttgttttactttttaaaatttctgtgagctgctctagaaaactaaaggacgaaaactttactgtcataattccaagttcagtcagggatttctcagaattgaggtgtgcagcatccagattcccctttatgtggatagggatccctgtgccatgtcttgcacttacctaagaactataggaattctccatgtacctcctacagtttttctagcagtgttggacaatggattctaaaggttcctgagactttgttaaatttctcataattccagagggaaggccaaaatattgagaatactcaatgataggatgagtttccactctacttccttatcctcaaggcacacaccagagttccactgggtgaggacagggaagtaggatgtcccaacaccctctgagggttttcatgcattaatcccgccatatgggctgatggttggaactgcctttagttctctaagtaaaggtctaaaaatgcacctgtggtttctgaacttgggtatacgctgatacataaggactaccatagaagttacatgccttaatcctgtaatacttttgtgtggtatcattctgctaatatattgtccacagggccaaaccccaagttacacagcgcaacagtacttgtcaaccactccatctcctcagtgacacaggtgctaaagtacctctcccctgaggcaaagtcccgacacatctgtggtaagtgcacataaacagaaatgggcagattttgaaagtgaatgcaaacaacttaattccaaaatacataaacatgacagaagaagtggttctctaacatatgccatgtttgatcaatataaagaataagtttttaaaatataaaagactttgatctccaagactaaatctagacttatctgcaaataagtaaattttcaaacagccaggggaaaatgcatttttttcaccgagtctcactaaatcattctgaattctggatcctgcttctcgtatcaccaattcctaatgttaggaatgtagaactgtctgctcttggggaaaaaaaaagcatctgtttttaattcaaagctctgggtatagaaaaactaattatggttttagctatctgtgtctgggtttataaaacatgcaccaatgtacactttctccttgtagattgaatgcaactatagaagtattagcataaaaatatgtggcctggaaggaatctctgaagatactgaagaacctcaagttccctacattgctaggagccaagggaaggagacactgtacacctagagcgctgaattagcagctgaggttttagtatttgaaagcaaataatataaagcgagtaatgtctacagtgggtctcagttaccatttggctacttatttaggactcgattaacttggcaacttttacaaaaaacattcacatcacaacatgcaacttaaaaaacagttaatgtaactatgccactgtcagcaaggccagcttgcataccagagttaagaatgagagtgtctgtctgcctagggcttaacattcaaagatatttataatctgtgttttaaggttaaattttatatgacccagttttccttctttgttcactatacactaaaattaaacgcctctacgctgtgcaagaaatcactatgtgtgattttactatttcaaccaatccatagaccctgaggatttggcagcagaattcaggagaaatgctacctaaagtgattgagctgttgctaattctaccttctgttccactcaagtacctccagggactaacaagggaaggcaagggcaactgtgactgactaggtaaccagctattctgttgtgacagaagaaaccaggtaatacttgattttcaaaagataattttaactgctgccctatactacttttagtatagtttggcttgaccttaatagccatgtccctcatcttagatagaataaccaaattggtttaaaattacttgatctatgtcactgaaacctgaaatatgccatcactaagagaacccccaaataaaaaataaagaactaaaaaacacaaccaaaccaaatcaaaccaaaaacctcattctctgtatcatactttaaaactaaaataaaaatccctgtgtcacaggtgcttgctcagggctgccaacttctatttttcacctgagagacatctaaaagcgcaaactatgcttgtaaaaaccaaaaagtaaatctctacataggacaatacttataagcagacctattgataccacttatatataattagtctgttttctttagaaagtatcagagcagaaacgtctttggttaattctttcctctacatgcaaaataaaatattcttaaacgatggactgtttatctctggatcttgatgagtttgtcaatgccatttagaaaaggggacaacacactagaaaagttgagataaaaatggaaggaaccaagaaagagagaaaacattcagttgccacattcccatcactgtcagttccaactgccagcagagaaatgccaataagaaataaaatcacacacacgtaccacagttgtagcttcatcagcttttccaatgattactactagcatatttccgactaaaggggtcaggatttaaagctagctacttttagcacaatttagctaatgcaacagaaatatgacaatttcttcattattcccccgaccccctgcaaaaaaagtgagatgaaaagaggaaagtagaatggcaatttttaagaaatgttttaaaaatctgtcagactcatcatcatcccagtttatccactctaactataaggagagaactatgtgattaacatgacaaatctctgaaccagtattacaagcatgtccctgtaattttttccctattaaaatctttttgaaatgaaaattaaataacctatcttggcttgttaaatactgcccacccttgcattgtacacagggaaggcaagaagactctgaggtgtcacatgccaagaacatagtttcagaaaatgaagataggcaaggcccaagtgtacatgaggcacacaatagaaaaggaatttcgccatctgtgatctcgaaattacaaatggagaatgacaaagaatgactctatataaggatatgtctctctatatatttataaatatttatataatttaccatgaagacatgcaagtagtgttatagcaactattatacaatataatacagaaggactgatcttccaatattacagttgctttagataaacagcaagtatgtcttatctattgcattcctctggagtgtttgaaactggagagaaattaagattccacactatgctacatttcttataagagacgttatatgcctcaatagtgttttgagtttgtttttttaaaaagctcaacacagataaagagaacaagagaagttcagtgcagcttcagggcagctttgatgcagcattagaagatgttcacttggggaggaaatgtattcctttcttttttttttgtttcccaattcaactgtattaggtttggcagcaaacacaaggtcaaacagaaagcacatatgtttgctagaaggcaaatttcaacagcaagcagaccaatttacctgaccttaataaggtctttacaacacaaaacacctagagagtataaaaacagcccattttaaaagtctggtagactttcatttgcctgattcctattagaagagtgagattagaacaaatatcttcctctttacagcttcgtaaattgagattgtatgaaaatcaggccaagaagcccaaatgttgaactaaaacacaggagaagcaggtaataaaacattaaaaaagaaatatttgcctaaatttatttccccagatattaattccttattggctaaatgtataaaatacaaagtttgaggattctaagcctcaataatatatctaatttatttctaaatctcaaatcacagtccaaagcattgtgcttccctcgtatcatcttggatgctgatattacaaacagttggaacccagaagacttaaggaagcagtctactctggtcagttttccttctactcaagtttctaaaggaggacacttaacagagatgaaagggcatcttctatcttgaaggctattaacccacactttctttctctccctaaacactaaagcctgcaaaatagctctagttagacttttctttcctttacctaactttcttatttttcataataaaaatgtaatatgttaagaactcttgctctaaaaaaaaaaaatcagggggacctaaaaaaaagtaattggatttgatagtacaactaggaccataaaataaaagcagagagattgaatcagacgagacatacaaaattttaaaaaaaaatctgaactccagggagggtactaggaatgaggcaaagtaaaggtgttcattctcaatacacgaaataaacacacaagccaaatatacatgaatactggctccctggcaacagacttcttatataatctaatatctgatcaatgactcttcagggtgggaaagttttgaatgaaaatatcaaacaagaagtttcacttttgctatataatctttgaattgaggcttaaaaaaattaggcaacccccctaaaattccattctatctcctatcctcaactcttttgtttcaaaggcagcttaaaaaatgagagctcattttaatgagtttctcccccttggatttttgctctatttttccttcttgtacaaagacattgattcctaatctacttgctgcctgccttaggtaattccttatcatgtattatgtcttcttataaataattgatcatgttactttcttttgcaagagaagatcaacactgatttttttacatagaaagtacagggacacacatgcatcaggtttaggaggaagatctcacacctttcaaagagatgcagcctggctcctatctgctgagtttactggctggcttactcttcccttggggggttttagtgctggctgagtggtggtggaggctgccggatcctttcaggccattcttgctgggtttgcaatgctcctgttggcaggacctcctggaggaggaagatcctgagtggctgggaggtgacttgcttctccccagatgtggggacgaactcctctggtcatggtggggccgtccagccctagatggtgaggaactagacgtgcgaggcaaggatgagcttcgaggagaggcactgggactcctgcgagggacaactggactcttgggtggtgtttttggattgtgaggagatcctggactcttgcactgagtagtgctccggggtttctgagatccattttgaagaatttgggccaggcgggagaaaaggtctgagtcggagttactactccctaggactttatatctgcgtagcctggcttctactccaggcctcgtgggtggctttcctggtggtggccgaggaaagaactgagacgaagttgagctattgacctgatctgtgttgacccatgaaactggccttggaattttgctctttctagactgggagatgatgggtgacagaaagctatcttcagctgacctactcaggtgagaatctactgtcagtcttgaaaagggagtgagcacttcctcctcacaaaagggagcaggaacagtagctagtttctcctctagcaatttatcagaggcacttgagaggtcgccaaggaaggacttgaattgtcttttttccaccagaagcttgactaggtctggctgataggctttcttttggaggagcttttcttttgcagaaactggagaggatgattccaaagttgagtctatctcttgtgctaaaacagggattcggctgtgtctagttacaaaggatgacctaaccatatccttccgggttggggcaccatgttcattctctgaaacacaatgaaatagttctccatttctaggggtgattttctctctcttgccctcttggtgcaaaaaagtagagaggtctccttgatgacctggcaagtcttcactcatgatgtcatcatccttagatatcttatttttttgcatttctgccacttggcctatctgaccttcaacatgtgggtcaatgtctctggaagaaatttctgaagttccaactgtcagaagcttcattatctcattatttttgtcttgatttggcaccacactaaaagtctgtgtttttgtcacatcaagaggttcagtagtagctgagtgatccttttccacaattaccaaatctcctgggagagaggagatctcaatacaatgctgccctctacttaacttctcatcttcattatctgactctaaaaggatgcttttctcttcagtttccccagggagattttcaaattctctcacaaccagtctattatgatcaggaagttcttttggtcccaggtcttgagatttgttactttctctaatgttgggtaacatgtcatgaccaatgtgatctatctgaagccccaaatctgttctgcttcctccactaggaggttcaccctctgtcacaaccaagccagagaagttttcccttggagagtaaagttccacagtgggctccatgggctgaagatctttcttctctggctgctgaccacagtgaaagcttcctgaagttgactgtgtagatgccacagaaggtctaggaattgtaatcgctgtaaggggtccttctgcctgcgcctccattagacttgtgggcgtcgctgcaataaactgactagcagctccaggctggagttccagcctatctgtatattgttctgaagcagcagtaggaggaccctctgcagaaagtgctaagaccacacctgaggtttccttctttaaatgatcattttctgcccaaggacctaactggagcttttcatcttgaggtgatgcctccaggacttgaagtacttcaggctcctcatcagaaggacttccagttgttttatgtcctacagcctcatttgtcctaaaatcctgaaggtcctgctccttgtccacaatcacccattctttggaatcaatttcttgcttgcaagagctcaggttaacagctataaatccattgctgccaccaccatctgcctgctcaggggtgttggcagaagcaggcttggaggcatctggaagatattcttcatcatagtgccagatgtggtcagtacgggacacagcaggaacgcaaggcttatgcagcagagcagggagaatagattcttttcctgcactggtatctttctgcattttctccaggcaggtctcaaggaacttgtcagtgtctggctttggctccagggtcagacgtttttccagctcaaagctgtgaatggaacgtaactttcgcaccagtggaatatctctgtctggctgagtaatctctgagcggacacgaattggtgacccaaggcttggagcattgagaagaccatttgcctggccatggctgttctcctcttcagtagcagccttacaaattccaagctttatcttgtttttgttggcatccatctcttcccaaacatccttctcctggggacgggggtgtcccagagatccaggcaatttatctggtgacacaccaacagggatgccattttctccatcgctaagctgttcatctggaaatacctcatctgtattttctcgaagcaagtctccagggatgggagtagcattggcaattccaattgcagcaggggtcaagcgagtgtgcaactgaggggtggtagaagtagtggtggttgttagggagccatcatttccagtcttctcccagtcaaaagggtcactctcaattactccaaaagtcttgatgctattgtcaaacacggatgtaagaagctggtagtctggttttgtaaaataatccaaagaagagatatggtctagaaagatgctgaattctggagggagatgtttcaacatgagcctgtggtcatatctctccttaatagagcctacttgctccttgtcctttatttttctccagggcagctgaccaaccacaaactccaccaacatgtagaataaggaccaaaggtcatcatgtcttcccatttccctgttccgatgtgcgttgattgatgcataacgaactgtccctcgaaaacctgccacagctcgaggtggtctgacgtcaccacaggaattggtaaattgtcgagccaagccaaaatcaagcatgtaacatttcctacatgtactaggaaagcgacccatagcgaagttcgacggtttgatgtctcgatgcaagaatcccacagaatgaatgctttcaatagactccaaaatctgtctacccagccggagagtggtactaatggtgaatgtgcctcgggactggctacggcgaagatctgccagattccgaccctgcaactgcatgaccacatagttgaatcgatcattcctcccacagccaataaatctacaaacatggtctttcccactttccatctttctttcactaggattccaacactcaggatatccagctgctctcctcccccactcattgcaatacactgatatggtagaacagctacacaggcatccagttcccaagggtggtttccatttaacctctactgtagcctcgacggatacaaaattaacttcgctgtagaataaagtatcctggcatcccaatggattatttacttctccgatttgacagaacatatacgtgagtcttttgtccctcccacagcatcccagggtgtcaacatcatctctgccacagcaaatgacgagcaaatccctcagatcattacttcagcaccctaagtacaagaaagtcgcggccttcactgtcgttacaacacagcaaacagattcagtagtcccatgttcctttccatgatagttggggaggcggggtgggaaataagcgctcagatttcctaggaatccttcgtgttcggtgctggtaccagaagtggcatgggtacaagtgatatgtgggtcacccacagagagagacgcagaacgaagcttcgtgaccctccaagttcagtgaagacacccaaagcctggggcaaaacgaggcggcagccttcggggaaatcgggcagaaccagaacgatctccgagatggagagtgacggggtctggcacgagccccgggcttgcagcgaactgaaagtccccggtacccctcccctcctcagcaggctcggtcactcggcgaggggtgcggccggaggagggggtcgagactgggggagggcggcgccctggggggtcggggggtgtgtcctacctgggccgtggcggacgcaggggtttctggaggagggctctggtccagctcaggaccgggaccggcgggggttaaccctcggcaggcgggaccgccactgcctgcccatcccccaccgccgactgcggcgggacccgagcgcggcttccagggccggccggctgggtagtcccctggggtaccgtccgcgtttactggcggcggcggcggcggctgctgctgctgttactgctgctgccggctcccccaagccgctgctcttgtgccagcacctgctccccctcctgccgccgccgccgcctcgtccccaccgctcccatcgccgctgcggcgactactgcagagcccgctgacccgacccgacgttattctcc

SEQ ID NO: 15440 - RNA, 9118 nt, Homo sapiens
  source 1..9118: mol_type = other RNA
gctgggattacaggcatgagccactgcgcctggccttgttttactttttaaaatttctgtgagctgctctagaaaactaaaggacgaaaactttactgtcataattccaagttcagtcagggatttctcagaattgaggtgtgcagcatccagattcccctttatgtggatagggatccctgtgccatgtcttgcacttacctaagaactataggaattctccatgtacctcctacagtttttctagcagtgttggacaatggattctaaaggttcctgagactttgttaaatttctcataattccagagggaaggccaaaatattgagaatactcaatgataggatgagtttccactctacttccttatcctcaaggcacacaccagagttccactgggtgaggacagggaagtaggatgtcccaacaccctctgagggttttcatgcattaatcccgccatatgggctgatggttggaactgcctttagttctctaagtaaaggtctaaaaatgcacctgtggtttctgaacttgggtatacgctgatacataaggactaccatagaagttacatgccttaatcctgtaatacttttgtgtggtatcattctgctaatatattgtccacagggccaaaccccaagttacacagcgcaacagtacttgtcaaccactccatctcctcagtgacacaggtgctaaagtacctctcccctgaggcaaagtcccgacacatctgtggtaagtgcacataaacagaaatgggcagattttgaaagtgaatgcaaacaacttaattccaaaatacataaacatgacagaagaagtggttctctaacatatgccatgtttgatcaatataaagaataagtttttaaaatataaaagactttgatctccaagactaaatctagacttatctgcaaataagtaaattttcaaacagccaggggaaaatgcatttttttcaccgagtctcactaaatcattctgaattctggatcctgcttctcgtatcaccaattcctaatgttaggaatgtagaactgtctgctcttggggaaaaaaaaagcatctgtttttaattcaaagctctgggtatagaaaaactaattatggttttagctatctgtgtctgggtttataaaacatgcaccaatgtacactttctccttgtagattgaatgcaactatagaagtattagcataaaaatatgtggcctggaaggaatctctgaagatactgaagaacctcaagttccctacattgctaggagccaagggaaggagacactgtacacctagagcgctgaattagcagctgaggttttagtatttgaaagcaaataatataaagcgagtaatgtctacagtgggtctcagttaccatttggctacttatttaggactcgattaacttggcaacttttacaaaaaacattcacatcacaacatgcaacttaaaaaacagttaatgtaactatgccactgtcagcaaggccagcttgcataccagagttaagaatgagagtgtctgtctgcctagggcttaacattcaaagatatttataatctgtgttttaaggttaaattttatatgacccagttttccttctttgttcactatacactaaaattaaacgcctctacgctgtgcaagaaatcactatgtgtgattttactatttcaaccaatccatagaccctgaggatttggcagcagaattcaggagaaatgctacctaaagtgattgagctgttgctaattctaccttctgttccactcaagtacctccagggactaacaagggaaggcaagggcaactgtgactgactaggtaaccagctattctgttgtgacagaagaaaccaggtaatacttgattttcaaaagataattttaactgctgccctatactacttttagtatagtttggcttgaccttaatagccatgtccctcatcttagatagaataaccaaattggtttaaaattacttgatctatgtcactgaaacctgaaatatgccatcactaagagaacccccaaataaaaaataaagaactaaaaaacacaaccaaaccaaatcaaaccaaaaacctcattctctgtatcatactttaaaactaaaataaaaatccctgtgtcacaggtgcttgctcagggctgccaacttctatttttcacctgagagacatctaaaagcgcaaactatgcttgtaaaaaccaaaaagtaaatctctacataggacaatacttataagcagacctattgataccacttatatataattagtctgttttctttagaaagtatcagagcagaaacgtctttggttaattctttcctctacatgcaaaataaaatattcttaaacgatggactgtttatctctggatcttgatgagtttgtcaatgccatttagaaaaggggacaacacactagaaaagttgagataaaaatggaaggaaccaagaaagagagaaaacattcagttgccacattcccatcactgtcagttccaactgccagcagagaaatgccaataagaaataaaatcacacacacgtaccacagttgtagcttcatcagcttttccaatgattactactagcatatttccgactaaaggggtcaggatttaaagctagctacttttagcacaatttagctaatgcaacagaaatatgacaatttcttcattattcccccgaccccctgcaaaaaaagtgagatgaaaagaggaaagtagaatggcaatttttaagaaatgttttaaaaatctgtcagactcatcatcatcccagtttatccactctaactataaggagagaactatgtgattaacatgacaaatctctgaaccagtattacaagcatgtccctgtaattttttccctattaaaatctttttgaaatgaaaattaaataacctatcttggcttgttaaatactgcccacccttgcattgtacacagggaaggcaagaagactctgaggtgtcacatgccaagaacatagtttcagaaaatgaagataggcaaggcccaagtgtacatgaggcacacaatagaaaaggaatttcgccatctgtgatctcgaaattacaaatggagaatgacaaagaatgactctatataaggatatgtctctctatatatttataaatatttatataatttaccatgaagacatgcaagtagtgttatagcaactattatacaatataatacagaaggactgatcttccaatattacagttgctttagataaacagcaagtatgtcttatctattgcattcctctggagtgtttgaaactggagagaaattaagattccacactatgctacatttcttataagagacgttatatgcctcaatagtgttttgagtttgtttttttaaaaagctcaacacagataaagagaacaagagaagttcagtgcagcttcagggcagctttgatgcagcattagaagatgttcacttggggaggaaatgtattcctttcttttttttttgtttcccaattcaactgtattaggtttggcagcaaacacaaggtcaaacagaaagcacatatgtttgctagaaggcaaatttcaacagcaagcagaccaatttacctgaccttaataaggtctttacaacacaaaacacctagagagtataaaaacagcccattttaaaagtctggtagactttcatttgcctgattcctattagaagagtgagattagaacaaatatcttcctctttacagcttcgtaaattgagattgtatgaaaatcaggccaagaagcccaaatgttgaactaaaacacaggagaagcaggtaataaaacattaaaaaagaaatatttgcctaaatttatttccccagatattaattccttattggctaaatgtataaaatacaaagtttgaggattctaagcctcaataatatatctaatttatttctaaatctcaaatcacagtccaaagcattgtgcttccctcgtatcatcttggatgctgatattacaaacagttggaacccagaagacttaaggaagcagtctactctggtcagttttccttctactcaagtttctaaaggaggacacttaacagagatgaaagggcatcttctatcttgaaggctattaacccacactttctttctctccctaaacactaaagcctgcaaaatagctctagttagacttttctttcctttacctaactttcttatttttcataataaaaatgtaatatgttaagaactcttgctctaaaaaaaaaaaatcagggggacctaaaaaaaagtaattggatttgatagtacaactaggaccataaaataaaagcagagagattgaatcagacgagacatacaaaattttaaaaaaaaatctgaactccagggagggtactaggaatgaggcaaagtaaaggtgttcattctcaatacacgaaataaacacacaagccaaatatacatgaatactggctccctggcaacagacttcttatataatctaatatctgatcaatgactcttcagggtgggaaagttttgaatgaaaatatcaaacaagaagtttcacttttgctatataatctttgaattgaggcttaaaaaaattaggcaacccccctaaaattccattctatctcctatcctcaactcttttgtttcaaaggcagcttaaaaaatgagagctcattttaatgagtttctcccccttggatttttgctctatttttccttcttgtacaaagacattgattcctaatctacttgctgcctgccttaggtaattccttatcatgtattatgtcttcttataaataattgatcatgttactttcttttgcaagagaagatcaacactgatttttttacatagaaagtacagggacacacatgcatcaggtttaggaggaagatctcacacctttcaaagagatgcagcctggctcctatctgctgagtttactggctggcttactcttcccttggggggttttagtgctggctgagtggtggtggaggctgccggatcctttcaggccattcttgctgggtttgcaatgctcctgttggcaggacctcctggaggaggaagatcctgagtggctgggaggtgacttgcttctccccagatgtggggacgaactcctctggtcatggtggggccgtccagccctagatggtgaggaactagacgtgcgaggcaaggatgagcttcgaggagaggcactgggactcctgcgagggacaactggactcttgggtggtgtttttggattgtgaggagatcctggactcttgcactgagtagtgctccggggtttctgagatccattttgaagaatttgggccaggcgggagaaaaggtctgagtcggagttactactccctaggactttatatctgcgtagcctggcttctactccaggcctcgtgggtggctttcctggtggtggccgaggaaagaactgagacgaagttgagctattgacctgatctgtgttgacccatgaaactggccttggaattttgctctttctagactgggagatgatgggtgacagaaagctatcttcagctgacctactcaggtgagaatctactgtcagtcttgaaaagggagtgagcacttcctcctcacaaaagggagcaggaacagtagctagtttctcctctagcaatttatcagaggcacttgagaggtcgccaaggaaggacttgaattgtcttttttccaccagaagcttgactaggtctggctgataggctttcttttggaggagcttttcttttgcagaaactggagaggatgattccaaagttgagtctatctcttgtgctaaaacagggattcggctgtgtctagttacaaaggatgacctaaccatatccttccgggttggggcaccatgttcattctctgaaacacaatgaaatagttctccatttctaggggtgattttctctctcttgccctcttggtgcaaaaaagtagagaggtctccttgatgacctggcaagtcttcactcatgatgtcatcatccttagatatcttatttttttgcatttctgccacttggcctatctgaccttcaacatgtgggtcaatgtctctggaagaaatttctgaagttccaactgtcagaagcttcattatctcattatttttgtcttgatttggcaccacactaaaagtctgtgtttttgtcacatcaagaggttcagtagtagctgagtgatccttttccacaattaccaaatctcctgggagagaggagatctcaatacaatgctgccctctacttaacttctcatcttcattatctgactctaaaaggatgcttttctcttcagtttccccagggagattttcaaattctctcacaaccagtctattatgatcaggaagttcttttggtcccaggtcttgagatttgttactttctctaatgttgggtaacatgtcatgaccaatgtgatctatctgaagccccaaatctgttctgcttcctccactaggaggttcaccctctgtcacaaccaagccagagaagttttcccttggagagtaaagttccacagtgggctccatgggctgaagatctttcttctctggctgctgaccacagtgaaagcttcctgaagttgactgtgtagatgccacagaaggtctaggaattgtaatcgctgtaaggggtccttctgcctgcgcctccattagacttgtgggcgtcgctgcaataaactgactagcagctccaggctggagttccagcctatctgtatattgttctgaagcagcagtaggaggaccctctgcagaaagtgctaagaccacacctgaggtttccttctttaaatgatcattttctgcccaaggacctaactggagcttttcatcttgaggtgatgcctccaggacttgaagtacttcaggctcctcatcagaaggacttccagttgttttatgtcctacagcctcatttgtcctaaaatcctgaaggtcctgctccttgtccacaatcacccattctttggaatcaatttcttgcttgcaagagctcaggttaacagctataaatccattgctgccaccaccatctgcctgctcaggggtgttggcagaagcaggcttggaggcatctggaagatattcttcatcatagtgccagatgtggtcagtacgggacacagcaggaacgcaaggcttatgcagcagagcagggagaatagattcttttcctgcactggtatctttctgcattttctccaggcaggtctcaaggaacttgtcagtgtctggctttggctccagggtcagacgtttttccagctcaaagctgtgaatggaacgtaactttcgcaccagtggaatatctctgtctggctgagtaatctctgagcggacacgaattggtgacccaaggcttggagcattgagaagaccatttgcctggccatggctgttctcctcttcagtagcagccttacaaattccaagctttatcttgtttttgttggcatccatctcttcccaaacatccttctcctggggacgggggtgtcccagagatccaggcaatttatctggtgacacaccaacagggatgccattttctccatcgctaagctgttcatctggaaatacctcatctgtattttctcgaagcaagtctccagggatgggagtagcattggcaattccaattgcagcaggggtcaagcgagtgtgcaactgaggggtggtagaagtagtggtggttgttagggagccatcatttccagtcttctcccagtcaaaagggtcactctcaattactccaaaagtcttgatgctattgtcaaacacggatgtaagaagctggtagtctggttttgtaaaataatccaaagaagagatatggtctagaaagatgctgaattctggagggagatgtttcaacatgagcctgtggtcatatctctccttaatagagcctacttgctccttgtcctttatttttctccagggcagctgaccaaccacaaactccaccaacatgtagaataaggaccaaaggtcatcatgtcttcccatttccctgttccgatgtgcgttgattgatgcataacgaactgtccctcgaaaacctgccacagctcgaggtggtctgacgtcaccacaggaattggtaaattgtcgagccaagccaaaatcaagcatgtaacatttcctacatgtactaggaaagcgacccatagcgaagttcgacggtttgatgtctcgatgcaagaatcccacagaatgaatgctttcaatagactccaaaatctgtctacccagccggagagtggtactaatggtgaatgtgcctcgggactggctacggcgaagatctgccagattccgaccctgcaactgcatgaccacatagttgaatcgatcattcctcccacagccaataaatctacaaacatggtctttcccttgcagctttttcaaaacagcaacttccattttcagaacttgttttggttgttgagctgattccaccttcagtgcaacattttccctggtgagcatgtccaaggcatcgtaaatttctccaaagcccccacccccaatctttctcaacactttccatctttctttcactaggattccaacactcaggatatccagctgctctcctcccccactcattgcaatacactgatatggtagaacagctacacaggcatccagttcccaagggtggtttccatttaacctgggccgtggcggacgcaggggtttctggaggagggctctggtccagctcaggaccgggaccggcgggggttaaccctcggcaggcgggaccgccactgcctgcccatcccccaccgccgactgcggcgggacccgagcgcggcttccagggccggccggctgggtagtcccctggggtaccgtccgcgtttactggcggcggcggcggcggctgctgctgctgttactgctgctgccggctcccccaagccgctgctcttgtgccagcacctgctccccctcctgccgccgccgccgcctcgtccccaccgctcccatcgccgctgcggcgactactgc

SEQ ID NO: 15441 - RNA, 4482 nt, Homo sapiens
  source 1..4482: mol_type = other RNA
gctgggattacaggcatgagccactgcgcctggcctttgccattacttttaatggcaaaaaatgcagttaacttttacaccaacctaatagaacgtaaagcagcttaaaacaagctgccctgactcagcagttcccaacaacaatcattcatctagaactacccaaggaaagcaacaaaaactttaattcccttaaggtttagaaccaatacaatgctcaaaggtctctgtgcaggaaaaaaaaatgcacagcaaaaagaaaaccttgctaggtacggtcgcttatgtctataatcccagcactttgggaggcccaggcgggagaactgcttgaggtgaggagttaggagatcagtatgggtaacacagtgtgactccatctccacgcgcaaatttttttttaattagttggacatggcgacgcatggctgtagtcccagatactcaggaggctgaggccagaggatcacttgagcccaggaggtcgaggctgcagtgagctatgattgtgccactgtacttcagcctgcgagacagagtaagaccttctctcttaaaacaaagtcacaggttctgagggttagggaaaaaataataaatttaataaagaaaaaagaaaactcaaaaaacaaacagcatttgcttcctatgaaatatttacccctttaccctaaatttaactgctttccagtccaaagctctacacacttcatgtgggcctttataaagcaaccactggctttatgatttgtctagaatacttgaagaaggaagtttatgactttgtcaaaaagctgttgtatattcccacttaacggataaataaagcaggttctattcaattggaagaaacaggaataaagacgtgtgcattttcagatttcctttgagtgccctggccttcagaccattcagtgtggcatttaactagtttagattatggttattgttgatcctctatttactgatgttccatgccttttatgaagaaaaatagctacctaattctctttcacccagtgaactatatattagagttgttgttgtttaattggaacagaaaaatagtttgatgaacaagctctatttttcttacccccaaattaattaccatcacttcaaggaagagagagggcaccaactctatttggaagctattttacgatctagactcccccacacacagtatcataggtgtctcatgtggatcacagaacacaggcaacataacaccagttgtagaggaaaagcctggcagagattccaagaacagcttgtctggggagtcctatggcagtaggccaagcaggaagaccatcgcggtaccttctggatggaggtactttcaaaccgggaggcccatccacatttcagattccactggagttctaagacctggtgtaacaggttctggtagccaacgacaatcccagcctaaaagtaggatttggcaatacagataacattcactctcttctggggcctagcaactcttcaacttttatctgtagtaaaaacagatgccaaatattttagctaacctggaatcaatgaaatatcttctcttacacttgtaccactactaataaggaaaacagataaaggggcatatgcattagatggtaccacagaaccctgaattcaactcggacccaagcaaaaattgaagccatcatcctgattataaaacccagtgagcttgatgcagaaagccactcctctctaggaataatcatgtcctatcacatagggactagcagcaagactgatttatccatgctaacggagggtataaatactcaaacccagaaaaaaactctggtatctgactccaggtctaaaggccagttgcccagggcatacaccacttacacagaaatgggtttccaaaggctacattgaacagccccacatctgctaggggatatgaaactgttcaggtccataggggctgaggtgttgcttgttttgcctcagctttccctaagctttcactgaccagctatcataggtatgagcgtggggacctaagttcaacctggctagagagcaggcaagccttcttaaagcgcagaggctccacagtcattagctaaggcagcaacgcctcctgctcaccagtgttggggaagagacttttgccttaggccagctgattgattacagtagttgggccaagtcctgaactgcatttccacaatgcaataataactactgcaagcaagccattatctggctaatttcctaaaattaaaaaaaaattttgttgttgggtgtggtaagggaggggtggtcctcactatgttgcccaggctggtcttgaactcctggcctcaagtcatcttcccactttggctaagtgctgtaattacaggcatgagccactgtgctcagccctaaaatattgttagagaacatttacagacataaagatgagctcagtctcatccttatcaatctcctaaaaggaaaatttaagatctagtacttataatcctgtcctcaaagcaaacctaaaaataactgtctctctgatttgttttacagaatcatttatagttgtgtctgtcaaatagcaagaatcattcctagccagtgatgtggttatcacttatcttatgtgagggtaaacctgcaatatcttagagtcctttctaaaattatacagaagtcaaaataacctttccaaaaaggagtactaaaaaactgtcactgatagaaaacatcaactgtatgccaaagtactaaaaaacaggcaatcattccatttcagttgtattcacctattttcatcagtaggcagggcagtgctatcagaagagtaggctgcccttctatgacgacagaagctgttcctgatacttagttctgccttgcacatagtagactcaggtatcagtaaaatgaatgaatgaattatgaaatacactgactggtgagtcagacgttttttaacattccaggaaaaaaaagaaggctgaaattcctaatgaaaaaaggatgtctcattgagagatttttgcattactctttctgtatacgaaagcttgttgtttagataaattaccacaacacaggactttcacatacctgtctttattttgcttttatttgtgatttgatttaaataaataagaaggttcacacaggttaataaaaagacaagcaagtttgttgtatggctgagaaataatatgctctcttggtgtatactgatggcattatcggataacaccatgaggaccctcctcttcctcatttcctgggtcagtcctggtcagtgcttcttccgcctagtgctccttttgtatcacttatgtacactggatggagagaaaagaactcttctatgccttagtcaacatagatagcagcaggtgagaaaaagagctgatttctgatgtaacagaagcagactgactcctgctagctccagatacaaaatgctctacaggatgacttactgtaagtcactactgataagttgtttgcgtgactgctgggagacagatttacagagttctgtgacagtctattctggtcttgctcagtttggtcaggagcaggagcccatgtgtcaggagcaggagcccatgtgtttttgctgatcgagtcgaactcggagcccccagggtcttttaagttgttttcatctgattgtcggttcttttggggagaggcaaaagggttgaagtttccttctaccttacgatgcggctgtgtgttgaactccgtttcaaaagatgacagctgctgcgttactcctaaaagtccacccacctccacactgagaatcacccagatgacatctccatagtagagtcctgtagcagtgcacatccgccactgtccctgatacattcctgctctgctggggctgcacatctggacgctgacatctgcaatctcttggggctctagcgatctcaccatcaccatgttcacatgtccaaattggtctcccccgacatatttaagacaaacccctggaggccaggcctctgccccagaattctggatccgccatgtttttacaaactgagtatccggaggtattgactccccttctcctatggtgacatcttcaacaaaggacatagagggcacactgatgtttgggctctcaaagtcataataggcgccaattgctgcttgtaggttccagttggtcatgtccaggaagaaggcgcaaccggcaggattgagctggaagccgagcagcctctggaactcggagatgagcacgtccttgtcggtggtgcccaggcagctgaacttctgcatcagctccgggtccaggtctacgtccatgccctccatggcggggaccggacacccgcttccccgcctcttcacaaccaagccgccgccgcgccgccgggcccggggacctggaggggggccgctgctagctagcttcgcgaccccgctcctttgaggtaggccccgggcctctcacagtctcataggggtaaactcact

SEQ ID NO: 15442 - RNA, 811 nt, Homo sapiens
  source 1..811: mol_type = other RNA
gctgggattacaggcatgagccactgcgcctggctaaaaccaatctttattaagcacctacttcatgccaagccctgggctagcttgttctcttaaggcctcacacctggtccaagaattctgaccacttgccggctgcaaggatttgggttagtgacttcacctcctacgtgttatatcctcttcatcccctgcctcatcttcctcacctggccttatggctttgccagtcaagcgagatgacacaagaaaggcatttactccataaatgcagctggtgcctttataaagaatcatgctatggctggcgtttatgaagcacacacgataccaggcacgatgctgagtgtcttcctcacagtaactccatgaatccatcgtctcgggcagaaggcacgcgtgcagaggcctggaggcttgctcttctcggctgctgagtagccagtagcctgacgcaaatccttatcagagcagaccacattttccagcccccgttcatgaagggtggagggagctgttgggaccggttctgagctcccatcagatcctctggagaactcctaggaatgcaggaggtggagctgaggggcagaggccagagctggactcctttccctgcactggatggtcagcgggccctttcctgaacgccaggcctcttgcagggcctacgtaggggctcctactgcggcttcttccctggcagagcccagcaggagctcctcggctcccctagctctgcttcctcttttgatttgcataacaatctgcccagacgagctttgtacctctgcatcagggctggagccca

SEQ ID NO: 15443 - RNA, 227 nt, Homo sapiens
  source 1..227: mol_type = other RNA
gctgggattacaggcatgagccactgcgcctggctcctcctctctcagaacattgggaggctgaagcaaggggttcacgagtactcctccccttcagtcaattcttttctacatagccgtgtccttcctttcagtctaagggtatcccagtctcagctgtacattaaagagaaggagtaggagaggtgtcaggatacagtggatgaagacaggctgagccaaagttc

SEQ ID NO: 15444 - RNA, 865 nt, Homo sapiens
  source 1..865: mol_type = other RNA
gctgggattacaggcatgagccactgcgcctggctgcacttttcttaaaatgaattaatgttcataaattctcacttccaacttagtaacattaatgagccacgtctgaatatttattttctacatatgatgcactctccacttctaaaatgtcatgatatggcatccttataattctactgatgactatataatattagttgatgtttggaatcaacagtttcaaatgatcctttatactgaaataagacacattattttacttcaattgtaattttagttccagagaaggcagtgctgtcttaaaggcttggacaagattttctttttctcttactccaggaagatcacttaacaacaaatatttgaggtttccatgtgatcaaatccaatgctcatgatacaagagtcggtggcgtcgatcgcctgaatcttgtatttgtccagagggcctgttggaaggtggttgtagtccttctgccacctctcctggccatggtagcgcaccatggccccacagcgcagcaaccactcggatgccgccctgtcagggccaacatccctgatgcgatcataatccaccttattaaacactgcattcaaccagccccagaagtatctggagtcacatgaccatgggagtttctttacgccacacaactgctgggaaatttttccaaacggcatcatttgatcatatgacccagcaattgtactcttgggcacttatcctagagaaacaaaaacaggttcacacaaaaggctgtacactcatgttcacagctgcttgattcacaatagctaaaaactagaaacaactcaaatgtccttcaatgagtgaacagttgaatgtacttgtattagt

SEQ ID NO: 15445 - RNA, 1432 nt, Homo sapiens
  source 1..1432: mol_type = other RNA
gctgggattacaggcatgagccactgcgcctggctgcacttttcttaaaatgaattaatgttcataaattctcacttccaacttagtaacattaatgagccacgtctgaatatttattttctacatatgatgcactctccacttctaaaatgtcatgatatggcatccttataattctactgatgactatataatattagttgatgtttggaatcaacagtttcaaatgatcctttatactgaaataagacacattattttacttcaattgtaattttagttccagagaaggcagtgctgtcttaaaggcttggacaagattttctttttctcttactccaggaagatcacttaacaacaaatatttgaggtttccatgtgatcaaatccaatgctcatgatacaagagtcggtggcgtcgatcgcctgaatcttgtatttgtccagagggcctgttggaaggtggttgtagtccttctgccacctctcctggccatggtagcgcaccatggccccacagcgcagcaaccactcggatgccgccctgtcagggccaacatccctgatgcgatcataatccaccttattaaacactgcattcaaccagccccagaagtatctggagtcacatgaccatgggagtttctttacgccacacaactgctgggaaatttttccaaacggcatcatttgatctgcacaggtgagtcgctgctcagagaccgcacagcacatttaaaactgtatctcggttcagtactcaagaaaaggacacagacttataaatggtggcaaaaaccgagctgtctggttcttccggtacccagtgccgggtcgagtacagagcaggcgctccatatttacaagacgaatcaatgactgaatgaatagcaccgccaggagccccataaaagaagtccagaagactgcgggctgtcagtcttcgctgtgacaaagagcctccgtgaggagcgaggattagggccggacagggagcgcccttctagtggacgctcgactgggctggggccgggatggagacggtgggtgcccaggccctccgtctaccgcgggccgcgtgcggggccgagcgaggacccggctggagctggagcgggggcggggcgggggcggggccgagggcgagccggaagaaagaagccgcagggcccgcccaaacaagaattttcaccgtaatcccgcccagagtttctcccacggccccatgtccgcatggcggtgaaggtcgaagacgcgcgacccaaagggccaggttttcagtcagcccagcgttggcgacgggcgagggcagaacacaaccaccaccctagtcccgcccggctcggggcctagcttctctactcacagcgtcggagggagggagggagggagcgagccagcgtccccgcgtctgcggcaccctggccggccc

SEQ ID NO: 15446 - RNA, 1410 nt, Homo sapiens
  source 1..1410: mol_type = other RNA
gctgggattacaggcatgagccactgcgcctggctgcacttttcttaaaatgaattaatgttcataaattctcacttccaacttagtaacattaatgagccacgtctgaatatttattttctacatatgatgcactctccacttctaaaatgtcatgatatggcatccttataattctactgatgactatataatattagttgatgtttggaatcaacagtttcaaatgatcctttatactgaaataagacacattattttacttcaattgtaattttagttccagagaaggcagtgctgtcttaaaggcttggacaagattttctttttctcttactccaggaagatcacttaacaacaaatatttgaggtttctatgactataatcgtgagtcaactgcaacaaaatggtcactgcaaatcatctgcattttctattagcaaaacgatagggtagttacccatgtgatcaaatccaatgctcatgatacaagagtcggtggcgtcgatcgcctgaatcttgtatttgtccagagggcctgttggaaggtggttgtagtccttctgccacctctcctggccatggtagcgcaccatggccccacagcgcagcaaccactcggatgccgccctgtcagggccaacatccctgatgcgatcataatccaccttattaaacactgcattcaaccagccccagaagtatctggagtcacatgaccatgggagtttctttacgccacacaactgctgggaaatttttccaaacggcatcatttgatctggttgtgatatggtactagttttgcaagatgctaccactgggaagactgggtaaagggtacacagaatctctattcttacaattgcatggaaatccacaattacctcacaaagttgaataaccatctctttttttcatctgtgatggaacaagcaggcaatattctacattgttttaacaaataaagcaaactatgtaccactgttctggtggtaaaaccctttaaccataataaatgtcatcacgtagcaaatgcttcactgtgctaaacacctgctgaccttatctcgtgtaatccgctcaacggccctaagactagggagacactgctatcattcctagttcactgaggagggtctgaggcaaagaggtgaagtgatttcctggagctacctgaccaaagactggaaccaagattcttagaggcacacgaagtccttctggtaataaatctgtataattctatttgttatgttcagctgtcctaaccctaaaaattaaaaactgccatcaagcatacagaatgagtgttagcaacaccggcacagtgacaattttaaagagttagaaggtcctttagagattacacagcccatcgccctcatttttacataaagggaatcagg

SEQ ID NO: 15447 - RNA, 888 nt, Homo sapiens
  source 1..888: mol_type = other RNA
gctgggattacaggcatgagccactgcgcctggctgcacttttcttaaaatgaattaatgttcataaattctcacttccaacttagtaacattaatgagccacgtctgaatatttattttctacatatgatgcactctccacttctaaaatgtcatgatatggcatccttataattctactgatgactatataatattagttgatgtttggaatcaacagtttcaaatgatcctttatactgaaataagacacattattttacttcaattgtaattttagttccagagaaggcagtgctgtcttaaaggcttggacaagattttctttttctcttactccaggaagatcacttaacaacaaatatttgaggtttcttaaatgacgcaaagcaatgatgcctttgtctgtgatattcccacaggatattatttccatttccaatatggttttttgtaaattttcaagttgactaagtctcagcaaacagtcatcctcgatataatgacacttgcacagccttattttttcaacatgctctaggccctccatgtgatcaaatccaatgctcatgatacaagagtcggtggcgtcgatcgcctgaatcttgtatttgtccagagggcctgttggaaggtggttgtagtccttctgccacctctcctggccatggtagcgcaccatggccccacagcgcagcaaccactcggatgccgccctgtcagggccaacatccctgatgcgatcataatccaccttattaaacactgcattcaaccagccccagaagtatctggagtcacatgaccatgggagtttctttacgccacacaactgctgggaaatttttccaaacggcatcatttgatagttccacatggctggggagg

SEQ ID NO: 15448 - RNA, 969 nt, Homo sapiens
  source 1..969: mol_type = other RNA
gctgggattacaggcatgagccactgcgcctggctgcacttttcttaaaatgaattaatgttcataaattctcacttccaacttagtaacattaatgagccacgtctgaatatttattttctacatatgatgcactctccacttctaaaatgtcatgatatggcatccttataattctactgatgactatataatattagttgatgtttggaatcaacagtttcaaatgatcctttatactgaaataagacacattattttacttcaattgtaattttagttccagagaaggcagtgctgtcttaaaggcttggacaagattttctttttctcttactccaggaagatcacttaacaacaaatatttgaggtttcttaaatgacgcaaagcaatgatgcctttgtctgtgatattcccacaggatattatttccatttccaatatggttttttgtaaattttcaagttgactaagtctcagcaaacagtcatcctcgatataatgacacttgcacagccttattttttcaacatgctctaggccctccatgtgatcaaatccaatgctcatgatacaagagtcggtggcgtcgatcgcctgaatcttgtatttgtccagagggcctgttggaaggtggttgtagtccttctgccacctctcctggccatggtagcgcaccatggccccacagcgcagcaaccactcggatgccgccctgtcagggccaacatccctgatgcgatcataatccaccttattaaacactgcattcaaccagccccagaagtatctggagtcacatgaccatgggagtttctttacgccacacaactgctgggaaatttttccaaacggcatcatttgatcatatgacccagcaattgtactcttgggcacttatcagcgtcggagggagggagggagggagcgagccagcgtccccgcgtctgcggcaccctggccggccc

SEQ ID NO: 15449 - RNA, 1640 nt, Homo sapiens
  source 1..1640: mol_type = other RNA
gctgggattacaggcatgagccactgcgcctggctgcacttttcttaaaatgaattaatgttcataaattctcacttccaacttagtaacattaatgagccacgtctgaatatttattttctacatatgatgcactctccacttctaaaatgtcatgatatggcatccttataattctactgatgactatataatattagttgatgtttggaatcaacagtttcaaatgatcctttatactgaaataagacacattattttacttcaattgtaattttagttccagagaaggcagtgctgtcttaaaggcttggacaagattttctttttctcttactccaggaagatcacttaacaacaaatatttgaggtttcttaaatgacgcaaagcaatgatgcctttgtctgtgatattcccacaggatattatttccatttccaatatggttttttgtaaattttcaagttgactaagtctcagcaaacagtcatcctcgatataatgacacttgcacagccttattttttcaacatgctctaggccctccatgtgatcaaatccaatgctcatgatacaagagtcggtggcgtcgatcgcctgaatcttgtatttgtccagagggcctgttggaaggtggttgtagtccttctgccacctctcctggccatggtagcgcaccatggccccacagcgcagcaaccactcggatgccgccctgtcagggccaacatccctgatgcgatcataatccaccttattaaacactgcattcaaccagccccagaagtatctggagtcacatgaccatgggagtttctttacgccacacaactgctgggaaatttttccaaacggcatcatttgatcatatgacccagcaattgtactcttgggcacttatcctgcacaggtgagtcgctgctcagagaccgcacagcacatttaaaactgtatctcggttcagtactcaagaaaaggacacagacttataaatggtggcaaaaaccgagctgtctggttcttccggtacccagtgccgggtcgagtacagagcaggcgctccatatttacaagacgaatcaatgactgaatgaatagcaccgccaggagccccataaaagaagtccagaagactgcgggctgtcagtcttcgctgtgacaaagagcctccgtgaggagcgaggattagggccggacagggagcgcccttctagtggacgctcgactgggctggggccgggatggagacggtgggtgcccaggccctccgtctaccgcgggccgcgtgcggggccgagcgaggacccggctggagctggagcgggggcggggcgggggcggggccgagggcgagccggaagaaagaagccgcagggcccgcccaaacaagaattttcaccgtaatcccgcccagagtttctcccacggccccatgtccgcatggcggtgaaggtcgaagacgcgcgacccaaagggccaggttttcagtcagcccagcgttggcgacgggcgagggcagaacacaaccaccaccctagtcccgcccggctcggggcctagcttctctactcacagcgtcggagggagggagggagggagcgagccagcgtccccgcgtctgcggcaccctggccggccc

SEQ ID NO: 15450 - RNA, 1604 nt, Homo sapiens
  source 1..1604: mol_type = other RNA
gctgggattacaggcatgagccactgcgcctggctgcacttttcttaaaatgaattaatgttcataaattctcacttccaacttagtaacattaatgagccacgtctgaatatttattttctacatatgatgcactctccacttctaaaatgtcatgatatggcatccttataattctactgatgactatataatattagttgatgtttggaatcaacagtttcaaatgatcctttatactgaaataagacacattattttacttcaattgtaattttagttccagagaaggcagtgctgtcttaaaggcttggacaagattttctttttctcttactccaggaagatcacttaacaacaaatatttgaggtttcttaaatgacgcaaagcaatgatgcctttgtctgtgatattcccacaggatattatttccatttccaatatggttttttgtaaattttcaagttgactaagtctcagcaaacagtcatcctcgatataatgacacttgcacagccttattttttcaacatgctctaggccctccatgtgatcaaatccaatgctcatgatacaagagtcggtggcgtcgatcgcctgaatcttgtatttgtccagagggcctgttggaaggtggttgtagtccttctgccacctctcctggccatggtagcgcaccatggccccacagcgcagcaaccactcggatgccgccctgtcagggccaacatccctgatgcgatcataatccaccttattaaacactgcattcaaccagccccagaagtatctggagtcacatgaccatgggagtttctttacgccacacaactgctgggaaatttttccaaacggcatcatttgatctgcacaggtgagtcgctgctcagagaccgcacagcacatttaaaactgtatctcggttcagtactcaagaaaaggacacagacttataaatggtggcaaaaaccgagctgtctggttcttccggtacccagtgccgggtcgagtacagagcaggcgctccatatttacaagacgaatcaatgactgaatgaatagcaccgccaggagccccataaaagaagtccagaagactgcgggctgtcagtcttcgctgtgacaaagagcctccgtgaggagcgaggattagggccggacagggagcgcccttctagtggacgctcgactgggctggggccgggatggagacggtgggtgcccaggccctccgtctaccgcgggccgcgtgcggggccgagcgaggacccggctggagctggagcgggggcggggcgggggcggggccgagggcgagccggaagaaagaagccgcagggcccgcccaaacaagaattttcaccgtaatcccgcccagagtttctcccacggccccatgtccgcatggcggtgaaggtcgaagacgcgcgacccaaagggccaggttttcagtcagcccagcgttggcgacgggcgagggcagaacacaaccaccaccctagtcccgcccggctcggggcctagcttctctactcacagcgtcggagggagggagggagggagcgagccagcgtccccgcgtctgcggcaccctggccggccc

SEQ ID NO: 15451 - RNA, 1206 nt, Homo sapiens
  source 1..1206: mol_type = other RNA
gctgggattacaggcatgagccactgcgcctggctgcacttttcttaaaatgaattaatgttcataaattctcacttccaacttagtaacattaatgagccacgtctgaatatttattttctacatatgatgcactctccacttctaaaatgtcatgatatggcatccttataattctactgatgactatataatattagttgatgtttggaatcaacagtttcaaatgatcctttatactgaaataagacacattattttacttcaattgtaattttagttccagagaaggcagtgctgtcttaaaggcttggacaagattttctttttctcttactccaggaagatcacttaacaacaaatatttgaggtttcttaaatgacgcaaagcaatgatgcctttgtctgtgatattcccacaggatattatttccatttccaatatggttttttgtaaattttcaagttgactaagtctcagcaaacagtcatcctcgatataatgacacttgcacagccttattttttcaacatgctctaggccctccatgtgatcaaatccaatgctcatgatacaagagtcggtggcgtcgatcgcctgaatcttgtatttgtccagagggcctgttggaaggtggttgtagtccttctgccacctctcctggccatggtagcgcaccatggccccacagcgcagcaaccactcggatgccgccctgtcagggccaacatccctgatgcgatcataatccaccttattaaacactgcattcaaccagccccagaagtatctggagtcacatgaccatgggagtttctttacgccacacaactgctgggaaatttttccaaacggcatcatttgatctgcaggttcattcgttgtatttacgggccggaggaaaggcagtgtatagagtagaggtcgggagtagctctggctttgaacaacccgtccactttctgttgaactctgggctagttacttaacctccttaaaggctcagttgtgaattggaccttagtctctcctgtaggtggtcatttgaaggataaaaggacctagcacacagtataagcaatcaaatatgctctttataagctggagtctttggcgttgcttggaagatctgaatacagtcttaaatcagttcctggcacaccccgcatagtgttgcccccgtcggaggcagctcttatgctaat

SEQ ID NO: 15452 - RNA, 1488 nt, Homo sapiens
  source 1..1488: mol_type = other RNA
gctgggattacaggcatgagccactgcgcctggctgcacttttcttaaaatgaattaatgttcataaattctcacttccaacttagtaacattaatgagccacgtctgaatatttattttctacatatgatgcactctccacttctaaaatgtcatgatatggcatccttataattctactgatgactatataatattagttgatgtttggaatcaacagtttcaaatgatcctttatactgaaataagacacattattttacttcaattgtaattttagttccagagaaggcagtgctgtcttaaaggcttggacaagattttctttttctcttactccaggaagatcacttaacaacaaatatttgaggtttcttaaatgacgcaaagcaatgatgcctttgtctgtgatattcccacaggatattatttccatttccaatatggttttttgtaaattttcaagttgactaagtctcagcaaacagtcatcctcgatataatgacacttgcacagccttattttttcaacatgctctaggccctccatgtgatcaaatccaatgctcatgatacaagagtcggtggcgtcgatcgcctgaatcttgtatttgtccagagggcctgttggaaggtggttgtagtccttctgccacctctcctggccatggtagcgcaccatggccccacagcgcagcaaccactcggatgccgccctgtcagggccaacatccctgatgcgatcataatccaccttattaaacactgcattcaaccagccccagaagtatctggagtcacatgaccatgggagtttctttacgccacacaactgctgggaaatttttccaaacggcatcatttgatctggttgtgatatggtactagttttgcaagatgctaccactgggaagactgggtaaagggtacacagaatctctattcttacaattgcatggaaatccacaattacctcacaaagttgaataaccatctctttttttcatctgtgatggaacaagcaggcaatattctacattgttttaacaaataaagcaaactatgtaccactgttctggtggtaaaaccctttaaccataataaatgtcatcacgtagcaaatgcttcactgtgctaaacacctgctgaccttatctcgtgtaatccgctcaacggccctaagactagggagacactgctatcattcctagttcactgaggagggtctgaggcaaagaggtgaagtgatttcctggagctacctgaccaaagactggaaccaagattcttagaggcacacgaagtccttctggtaataaatctgtataattctatttgttatgttcagctgtcctaaccctaaaaattaaaaactgccatcaagcatacagaatgagtgttagcaacaccggcacagtgacaattttaaagagttagaaggtcctttagagattacacagcccatcgccctcatttttacataaaggg

SEQ ID NO: 15453 - RNA, 4237 nt, Homo sapiens
  source 1..4237: mol_type = other RNA
gctgggattacaggcatgagccactgcgcctggctgcacttttcttaaaatgaattaatgttcataaattctcacttccaacttagtaacattaatgagccacgtctgaatatttattttctacatatgatgcactctccacttctaaaatgtcatgatatggcatccttataattctactgatgactatataatattagttgatgtttggaatcaacagtttcaaatgatcctttatactgaaataagacacattattttacttcaattgtaattttagttccagagaaggcagtgctgtcttaaaggcttggacaagattttctttttctcttactccaggaagatcacttaacaacaaatatttgaggtttcttaaatgacgcaaagcaatgatgcctttgtctgtgatattcccacaggatattatttccatttccaatatggttttttgtaaattttcaagttgactaagtctcagcaaacagtcatcctcgatataatgacacttgcacagccttattttttcaacatgctctaggccctccatgtgatcaaatccaatgctcatgatacaagagtcggtggcgtcgatcgcctgaatcttgtatttgtccagagggcctgttggaaggtggttgtagtccttctgccacctctcctggccatggtagcgcaccatggccccacagcgcagcaaccactcggatgccgccctgtcagggccaacatccctgatgcgatcataatccaccttattaaacactgcattcaaccagccccagaagtatctggagtcacatgaccatgggagtttctttacgccacacaactgctgggaaatttttccaaacggcatcatttgatttgccactcaacaattactgagcaagtcactcctgtttcttgttcttggggttttttatttgtttgctgcaaaaaaatgaggggttggactggatggtgtctaaggctccttccggctagaacgttaagttccactgttgaaacctcaattggagtctgcctgtcgtactgccatctagtgtccattcaggcgctgtagctatgaatttgctgaagctggctcctctattccccatctatatttccagcatcaaaatgacagactaaaatcaccgaaagagcaacgtgtcaaggttaagatgcttgcatccaggaaagaagaggagacatgaaaatagatctacctatgacaaggctgcaagtggtgttaccagagcagtgtaaacaaaaaaactgttttaagggcagctgggaaagactgggcaagtaacttcacctctctgacctctggttttctcatttgtaaaatgagatgatttgcttaatttccagctgtcaaaatgtataaccataatttgagaaagtgattcctggagtaggtttcgatttgattgacctcaattcaagtttccctagtagtatgctaggtgtgtgcaggggactggatgtggcagggaggaggagatggggagacaaagataaatgaaacatggtgtttgctttgagcatctgacaatttaatgcaggatggagtgggctaagacacgttatcaagtagttaaaataagtgacagaacttgataaatgcctcaaaagagttaaaataaggacagaaaggatttcaacaaacaaaggtgccaggaaaaattatgccagattattagctgaagcaggaacatttaaggcatgttattttcagtttcactagcacatgtgagtcatgagaagaggcaggcaacttgcacagtcaggtcgtgaagtgttttgcatgctcagccagggaatttggactgtattctgtatgtagcagggagtcaccgaggtttctgaacaaagcactggccctttgggaggccgaggcaggcagatcacgaggtcaggatatcgagacgatcctggctaacacggtgaaactctgtctctactaaaaataccaaaaaataaaaaaataaaaaattagccaggcatggtggcatgcgcctgtagtcccagctactcgggaggctgaggcaggagaatcgcttgaacccgggaggcagagattgcagtaagctgagattgtaccagactgcactccagcgtggacaacagagtgagactccatctcaaaaataaataaataaataaaatagaacaaagcattggcattgttacggttgtgcttcaagaaattgactcagcagcatcaagattaagggtcaacagaatgggacagccagtcagcaagggcttcaatcacatgaggccatacgaaagggcctagttggggaaggatgggaatgacattacatagttagttccatatgactcagttaagtgagatgtaggggcaagggctagaggagttgaaaatgacaccaagttttggccctgggtcactggtagtaggatggtgatgccattaaaagaaatcacattaggagaacagggttataggttcagatttttttcttttagtttttcataatctacatactaagtgttagcaggatttctaagtgcagatgaccaacaaatcattggaatcagaggtcacaaaacattagagctgtaaggaatttagatcacctggatgaaatctctcatttagaggtgaggaaactgaagccctgatattaagtaacttcctgacatcctaaatcctttctgaaacaaggtggggtattaataaatgcatgtgtttaaagggacttgctcaatgtttcatgactaattggtggcagtgttgaaacctgaacccagttctctaccagcccagggtcctttcctcaatcattacatggttctggaattcaagagaaagaagaggactagaaagatgcctgagagggaaacaccttaaagctgaggaagtgattgaggatgctgaggccgtggaacagtgagagatgtgaactgaagacagaaccaactaccctttcatccctttttcactacagccgtcttcattactgcaagcctctgctccactacctcttatcatgttctcaaccctttccaactttttgttaaagcgctctctgcctgtgcccaccttgaataactctattagttgtcaatcttatttacaaatatgggctttcccagcttctactcaggctgttttctcttagcctccctcccccatcaccatcaatctgtggaaatcccacccaacctcaagaccttactcaaatgccatgtccattcattcattcgctcaaaaaatgtttattgaatgtctgctatacttagtgcaaaggcaacaatggtaagacaaaacaaacaaaaacaagaacaaaggagaaagagacacacagaaagacaaggttcctgacctcatagaacatataatttaataaagagagataacatataaagagataaataacacccaacgtggttggataatagaggtgtgaacaaataccatgagaatctagagaagggagtgagaagaaggccttcacactagaggtgtcttttgaaatgggtcttaatgattaagagttttcagttagtctagaagcagaagcagaatatgaaaaaaaaaattccagttagaacgaaaaaagagtatgcaaagtaaaagaacaaggatggcatcttattcatttccatttttctcagcataatgcaaaagtttaataaatatttgtttattaatagtcttcaacggttgacatgtttccatggagaaaggtaaaaccagttaaactgttattaagcaggtgaattagagtggtctttgaaaactgaatatttttgcttgattcattttggcccatcttataatttagcttaaacgaaaggccaaatttacttaggctgtaatctctaaaaacacaagatattagatttaaaatgttttaaacataaaaattaaatttatatttggcaatagaggtaacaaaaattggtaggtttttacatttcaactgcaactttgctaatgattttgcaaattattcctacttgagtccaaacagttgcctttgggaacgctttctatagggaaagaggagacctctagtgggaagttagtgaatctagctctaataaattaaaagaacccagttaaacgcaaattagaaaataaccactactaaattactgctgccatagataatccaccatgattgagtttcatacagggatgcacaaatggcttaacatacacaagtcaataaatgttatatgccacataaacacaattaaaaacaaaaatcac

SEQ ID NO: 15454 - RNA, 1648 nt, Homo sapiens
  source 1..1648: mol_type = other RNA
gctgggattacaggcatgagccactgcgcctggctgcacttttcttaaaatgaattaatgttcataaattctcacttccaacttagtaacattaatgagccacgtctgaatatttattttctacatatgatgcactctccacttctaaaatgtcatgatatggcatccttataattctactgatgactatataatattagttgatgtttggaatcaacagtttcaaatgatcctttatactgaaataagacacattattttacttcaattgtaattttagttccagagaaggcagtgctgtcttaaaggcttggacaagattttctttttctcttactccaggaagatcacttaacaacaaatatttgaggtttcttaacagcattatcaagtttccactttggctttgatcatctaccttaaatgacgcaaagcaatgatgcctttgtctgtgatattcccacaggatattatttccatttccaatatggttttttgtaaattttcaagttgactaagtctcagcaaacagtcatcctcgatataatgacacttgcacagccttattttttcaacatgctctaggccctccatgtgatcaaatccaatgctcatgatacaagagtcggtggcgtcgatcgcctgaatcttgtatttgtccagagggcctgttggaaggtggttgtagtccttctgccacctctcctggccatggtagcgcaccatggccccacagcgcagcaaccactcggatgccgccctgtcagggccaacatccctgatgcgatcataatccaccttattaaacactgcattcaaccagccccagaagtatctggagtcacatgaccatgggagtttctttacgccacacaactgctgggaaatttttccaaacggcatcatttgatctgcacaggtgagtcgctgctcagagaccgcacagcacatttaaaactgtatctcggttcagtactcaagaaaaggacacagacttataaatggtggcaaaaaccgagctgtctggttcttccggtacccagtgccgggtcgagtacagagcaggcgctccatatttacaagacgaatcaatgactgaatgaatagcaccgccaggagccccataaaagaagtccagaagactgcgggctgtcagtcttcgctgtgacaaagagcctccgtgaggagcgaggattagggccggacagggagcgcccttctagtggacgctcgactgggctggggccgggatggagacggtgggtgcccaggccctccgtctaccgcgggccgcgtgcggggccgagcgaggacccggctggagctggagcgggggcggggcgggggcggggccgagggcgagccggaagaaagaagccgcagggcccgcccaaacaagaattttcaccgtaatcccgcccagagtttctcccacggccccatgtccgcatggcggtgaaggtcgaagacgcgcgacccaaagggccaggttttcagtcagcccagcgttggcgacgggcgagggcagaacacaaccaccaccctagtcccgcccggctcggggcctagcttctctactcacagcgtcggagggagggagggagggagcgagccagcgtccccgcgtctgcggcaccctggccggccc

SEQ ID NO: 15455 - RNA, 1534 nt, Homo sapiens
  source 1..1534: mol_type = other RNA
gctgggattacaggcatgagccactgcgcctggctgcacttttcttaaaatgaattaatgttcataaattctcacttccaacttagtaacattaatgagccacgtctgaatatttattttctacatatgatgcactctccacttctaaaatgtcatgatatggcatccttataattctactgatgactatataatattagttgatgtttggaatcaacagtttcaaatgatcctttatactgaaataagacacattattttacttcaattgtaattttagttccagagaaggcagtgctgtcttaaaggcttggacaagattttctttttctcttactccaggaagatcacttaacaacaaatatttgaggtttcttaacagcattatcaagtttccactttggctttgatcatctaccttaaatgacgcaaagcaatgatgcctttgtctgtgatattcccacaggatattatttccatttccaatatggttttttgtaaattttcaagttgactaagtctcagcaaacagtcatcctcgatataatgacacttgcacagccttattttttcaacatgctctaggccctccatgtgatcaaatccaatgctcatgatacaagagtcggtggcgtcgatcgcctgaatcttgtatttgtccagagggcctgttggaaggtggttgtagtccttctgccacctctcctggccatggtagcgcaccatggccccacagcgcagcaaccactcggatgccgccctgtcagggccaacatccctgatgcgatcataatccaccttattaaacactgcattcaaccagccccagaagtatctggagtcacatgaccatgggagtttctttacgccacacaactgctgggaaatttttccaaacggcatcatttgatctggttgtgatatggtactagttttgcaagatgctaccactgggaagactgggtaaagggtacacagaatctctattcttacaattgcatggaaatccacaattacctcacaaagttgaataaccatctctttttttcatctgtgatggaacaagcaggcaatattctacattgttttaacaaataaagcaaactatgtaccactgttctggtggtaaaaccctttaaccataataaatgtcatcacgtagcaaatgcttcactgtgctaaacacctgctgaccttatctcgtgtaatccgctcaacggccctaagactagggagacactgctatcattcctagttcactgaggagggtctgaggcaaagaggtgaagtgatttcctggagctacctgaccaaagactggaaccaagattcttagaggcacacgaagtccttctggtaataaatctgtataattctatttgttatgttcagctgtcctaaccctaaaaattaaaaactgccatcaagcatacagaatgagtgttagcaacaccggcacagtgacaattttaaagagttagaaggtcctttagagattacacagcccatcgccctcatttttacataaagggaa

SEQ ID NO: 15456 - RNA, 5276 nt, Homo sapiens
  source 1..5276: mol_type = other RNA
gctgggattacaggcatgagccactgcgctggatctgctccacgttttttttttttaattatgtatttccacctgctatcccctctgctgggaatgccttttccttttcccagctttgcaaaatccttcccagccttcaaatatctgaggcaagcctgggcacagtggctcacacctataatcccagtatttggggaagcttaggtgggaggaccacttgagcccaggagtttgagaccagcctgggcaacacagcaagaccctgtctgtacaaattaaaaattaaaaaaaaaaattagctgggcatgttggtgcacacctgtgatcgcagctacttgggaggcccaggaggttgaggctgtggtgagctgtgattgcaccactgccctctagtctgggtgacagaatgagacctcatctcaaaagaaagaatctctgaggcgtcatctccattcattcattcattcattcattcattcattcaaatgcatattcatggaggatctgcaacatgccaggcacagcagccaccaggaatgaagcagtggctgggtgcagtggctcatgcctatagtcccagcattttgggaggctgaggcaggtggatctcttgtgcccgggagtttgagaccagccgggacaacatggtgaaaccccatctctacaaaaaatacaaaaattagccaggtgtggtggttctcatatgtagaaaacaataaaaataatttttaaagaaaggaatcaagcagtggatatgacaaaggccacgacacactctcaggtgaagccttccaacctttcgccagggcaatgcgagcccttctgctcagccactggaatctcttcctcaaagtctcccttgccacagtacacatgcatgggagaacatgcatgcacacacacatgcgcgcacacacacacatgcgcacacacatgtgcacacatacacacacaggcacatgcacgcacgcacatgcacgcacgcacatgcacacgtacacacatatgtgcacacacgcatggcttggtaggcttcacctgagagttatgaatgcaccattttccttggtgcattcataacactgtttgtgcctctcttttatttattttatttatttttattttttgagacagtctcactttgtcacccagcctggagtacagtggcatgatcccggctcactgcaacctctgactccagggttcaagcaattctctggcctcagcctcctaagtagctgggattacaggagcacaccaccatgcctggctaacttttgtatttttagtagaaacggggtttcatcatattggccaggctggtctcaaactcctgacctcatgatctgcccaccttggcctcccaaagtgctgagattacaggcgtgagccaccgcacccggcctgtgcctctcttttaacacttatattttgatattttctggattgtgaaagccctgttgggtgccttccttacccgtactacctctttttttcaggattcgcccaggacctgactaaaaccagtcctggcttagaaaacaaccatatctgtcaaaggaaagggaggtggagctgaggacagcgacgttcgttcggtgacagtattttctaaacctgatatgggggctcttattttaacaactctaagacaacagtgtctctaagggattttggacatggcctctgtcattctgcagctgcagtgagtccaaatagcaatcagaaaaggccaccagatgcagcccagtgggtgcccagcctggctggtagaagctggttccatccgagctcagctcttcccacccactaagcaagccccttcccgctccctccctccgtctcctctcccactgcacgagcccatcccccacctgaccctttcccccatctcctgcccaggccacagagcagggctgtcacactcacatgcctcccctgtctttttttgcaggtcaacctgtctgctctcagccaccgcaagctctaactcaacaacttcctctttgaaaatttcctctttgtcctcgggaaataccaactgccctggcccatgtgtgctcctgggctgtagcctgggctggtctcaaaggcagcaccattgagttctcccctctccacccaggccccacaggggaagtccctggctccaggcccctccttcactcactctcactggttcctcttggaggatggaaggggctcagcccctgggatggaagaggagacacagacaaactaaacctggaaacgtgcagtggggaagcgccagccagaccagtccccgagaccagggcaaacccctctccccctgcctctgttcgcaggagagcgcgcgcgcgcgcgcgtgtgtgtgtgtgtgtgtgtgtgtgtgtgagagagagagagagagagagagcgcacatgcatgtgtactgcagaaatggagacttcaaggaagggattaccatggctgagctgaagaactcatatttgggtcacacatacgatctttccatgaagcctggctttctttttcttttcttttttgagacaggggctcactctgttgcccaggctgaagtgcagtggtgcaatcacagctcacttcagactcgaactcctgggctcaagcgatcctcctgcctcaactttccaaagtgctgggattaaaggcaccagccactgtgctcaccctggcattctgtatggggctacagacagagttagattttctgctatgtccaccccatcagagcaaagatgacacgcacgttctcagcagtccctgtgtcccccatgcccaggttgaccctcttcagtctctgcaccacttcccacccccacaccgtctgtacccacaactacccctcccaagcatcgccaaatcctcagctcttgcacacaaaccacacccacgagtggacacacgcaggcactggggtttctgagaactacacccagccagaaactcggaggagaaaccgtgaggcctctggctgcctctgtccatggctggggagagtgtggtggtgtgggccagggccagcctacagtccatgtgccctgggaaagatcacaggcccgcctgagagcatgggctggtggccccacccagccatgctccaggctggcctggggggcccagagctaaaggtggttgcgggctgcccaggttccacagcccttgcagctacagggcaagggtgctttacaaagttaatcctaggagggagtttgccgggttctcttgtccttcttcccagactctggtcaacccagggtgggttctgggggaaaaggagaattgtcaaagaaatcacagggcagataagtttggccgatggagactcagcagccgtttccaggaacaagaaagagggggaaatggtgatggagataaataggggtggatgaggagggtttattcattcagtccacagacgttgagaggtgccagccctgccctgcccaggcgctagttgtgggtgctgggtgaggatggcagcaggaaatccagggctgagaagcctcatgaggattcagagtgaagaggtgggtgaggaggcaaggcgcggaggctcatgtctgtaatctcagcactttgggaggctgaggcaggtagatcacctgaggtcaggagtttgagaccagcctagccaacatggtgaaaccccatctctaccaaaaatacaaaaaagcagctgggcatggtggtgggtgcctgtaatctcagttactcgggaagctgaggcaggagaatcgcctgaacttaggaggcagaggttgcagtgaactgagatcgtgcattgcactccagcctgggcgacaaagcgaaactctgtctcaaaagaaaaaaaaaaaggagattcgggtgaggatcagggtgccgggtggaaacatgggagcgagggggcagtgggatggtgagagggaaggtgctggaggctggctgagattccggcctccagcctcactattcaccgacacttaaggggcagccccgtctcccccttcgggctcatcaggagctggggcgtccacagccccatcctcactggccaccagtggctcctcctcccctttgaggctggggcctgacccagacttcagctcctccatcgccagggagccctggcgagacttccgtctgccaaagaaagtggtgagcgtgggccgacggctagacccctccccatcggggaacccagagcccttgtcgcccccggaccctcccacggtcactgtcacggccccctcctcagggacctgggctggcccagcccaggcgtccaccaccccgttacgcttgccgcctctgctcagcacgagggccccagtccgccgcttctgccgccggcgccacagcaggagcagagccacgaggactatgaccgccagcagggccacaagcacagccactggcagcatgcctcgtgagttctcatctgggttccggaagggcacagtgcttgcgttggtggaggtcgttggagacatcattgtagatagttttacgctagagacctggggtccactggccccgctggagggctccagagagccagttgtcatggtaacagggggtccagtggtcccagtggaggtctccagagagtcagttgccatggtaacagggggtccagaggtgcctttggaagtctccagagagacagttgccatggtaagagggggtccagaggtgcctctggaggtctccagagagctagctgccgtggtaacaggggctccactggtcctactggaggtttctggagagttcgttgttatggttccacctgtcacggtgtgggatcctagagagtttgctgttatgggaacagcaggatgactggttgcatgaggggtttcctggggcactgatgacatcttgatggaaacttcctggtaggttgttggctcaggtaaaggggaaccagtgctggcaccaatggaagtccaaagaggggatccctcattgatggaagttgagggaggtagggctgaggtctggtccccagtgctgtcggccttagggtcacttgttattgaagtggtgtacatctttgagctcaggggctcgctagtagagaccaaaggctctccggaggtgggtgtctgcactgctgttgtgctccccagagcgtctgggcttaccaccagcaccccaaggagaaggagaagcgtggccatttccaggcaaacaggcaggagcaagagctgggaccggctcggctgataaggacgcagcactggggccaggtcactccaccacctcccgaggctggggcaagact

SEQ ID NO: 15457 - RNA, 5324 nt, Homo sapiens
  source 1..5324: mol_type = other RNA
gctgggattacaggcatgagccactgcgctggatctgctccacgttttttttttttaattatgtatttccacctgctatcccctctgctgggaatgccttttccttttcccagctttgcaaaatccttcccagccttcaaatatctgaggcaagcctgggcacagtggctcacacctataatcccagtatttggggaagcttaggtgggaggaccacttgagcccaggagtttgagaccagcctgggcaacacagcaagaccctgtctgtacaaattaaaaattaaaaaaaaaaattagctgggcatgttggtgcacacctgtgatcgcagctacttgggaggcccaggaggttgaggctgtggtgagctgtgattgcaccactgccctctagtctgggtgacagaatgagacctcatctcaaaagaaagaatctctgaggcgtcatctccattcattcattcattcattcattcattcattcaaatgcatattcatggaggatctgcaacatgccaggcacagcagccaccaggaatgaagcagtggctgggtgcagtggctcatgcctatagtcccagcattttgggaggctgaggcaggtggatctcttgtgcccgggagtttgagaccagccgggacaacatggtgaaaccccatctctacaaaaaatacaaaaattagccaggtgtggtggttctcatatgtagaaaacaataaaaataatttttaaagaaaggaatcaagcagtggatatgacaaaggccacgacacactctcaggtgaagccttccaacctttcgccagggcaatgcgagcccttctgctcagccactggaatctcttcctcaaagtctcccttgccacagtacacatgcatgggagaacatgcatgcacacacacatgcgcgcacacacacacatgcgcacacacatgtgcacacatacacacacaggcacatgcacgcacgcacatgcacgcacgcacatgcacacgtacacacatatgtgcacacacgcatggcttggtaggcttcacctgagagttatgaatgcaccattttccttggtgcattcataacactgtttgtgcctctcttttatttattttatttatttttattttttgagacagtctcactttgtcacccagcctggagtacagtggcatgatcccggctcactgcaacctctgactccagggttcaagcaattctctggcctcagcctcctaagtagctgggattacaggagcacaccaccatgcctggctaacttttgtatttttagtagaaacggggtttcatcatattggccaggctggtctcaaactcctgacctcatgatctgcccaccttggcctcccaaagtgctgagattacaggcgtgagccaccgcacccggcctgtgcctctcttttaacacttatattttgatattttctggattgtgaaagccctgttgggtgccttccttacccgtactacctctttttttcaggattcgcccaggacctgactaaaaccagtcctggcttagaaaacaaccatatctgtcaaaggaaagggaggtggagctgaggacagcgacgttcgttcggtgacagtattttctaaacctgatatgggggctcttattttaacaactctaagacaacagtgtctctaagggattttggacatggcctctgtcattctgcagctgcagtgagtccaaatagcaatcagaaaaggccaccagatgcagcccagtgggtgcccagcctggctggtagaagctggttccatccgagctcagctcttcccacccactaagcaagccccttcccgctccctccctccgtctcctctcccactgcacgagcccatcccccacctgaccctttcccccatctcctgcccaggccacagagcagggctgtcacactcacatgcctcccctgtctttttttgcaggtcaacctgtctgctctcagccaccgcaagctctaactcaacaacttcctctttgaaaatttcctctttgtcctcgggaaataccaactgccctggcccatgtgtgctcctgggctgtagcctgggctggtctcaaaggcagcaccattgagttctcccctctccacccaggccccacaggggaagtccctggctccaggcccctccttcactcactctcactggttcctcttggaggatggaaggggctcagcccctgggatggaagaggagacacagacaaactaaacctggaaacgtgcagtggggaagcgccagccagaccagtccccgagaccagggcaaacccctctccccctgcctctgttcgcaggagagcgcgcgcgcgcgcgcgtgtgtgtgtgtgtgtgtgtgtgtgtgtgagagagagagagagagagagagcgcacatgcatgtgtactgcagaaatggagacttcaaggaagggattaccatggctgagctgaagaactcatatttgggtcacacatacgatctttccatgaagcctggctttctttttcttttcttttttgagacaggggctcactctgttgcccaggctgaagtgcagtggtgcaatcacagctcacttcagactcgaactcctgggctcaagcgatcctcctgcctcaactttccaaagtgctgggattaaaggcaccagccactgtgctcaccctggcattctgtatggggctacagacagagttagattttctgctatgtccaccccatcagagcaaagatgacacgcacgttctcagcagtccctgtgtcccccatgcccaggttgaccctcttcagtctctgcaccacttcccacccccacaccgtctgtacccacaactacccctcccaagcatcgccaaatcctcagctcttgcacacaaaccacacccacgagtggacacacgcaggcactggggtttctgagaactacacccagccagaaactcggaggagaaaccgtgaggcctctggctgcctctgtccatggctggggagagtgtggtggtgtgggccagggccagcctacagtccatgtgccctgggaaagatcacaggcccgcctgagagcatgggctggtggccccacccagccatgctccaggctggcctggggggcccagagctaaaggtggttgcgggctgcccaggttccacagcccttgcagctacagggcaagggtgctttacaaagttaatcctaggagggagtttgccgggttctcttgtccttcttcccagactctggtcaacccagggtgggttctgggggaaaaggagaattgtcaaagaaatcacagggcagataagtttggccgatggagactcagcagccgtttccaggaacaagaaagagggggaaatggtgatggagataaataggggtggatgaggagggtttattcattcagtccacagacgttgagaggtgccagccctgccctgcccaggcgctagttgtgggtgctgggtgaggatggcagcaggaaatccagggctgagaagcctcatgaggattcagagtgaagaggtgggtgaggaggcaaggcgcggaggctcatgtctgtaatctcagcactttgggaggctgaggcaggtagatcacctgaggtcaggagtttgagaccagcctagccaacatggtgaaaccccatctctaccaaaaatacaaaaaagcagctgggcatggtggtgggtgcctgtaatctcagttactcgggaagctgaggcaggagaatcgcctgaacttaggaggcagaggttgcagtgaactgagatcgtgcattgcactccagcctgggcgacaaagcgaaactctgtctcaaaagaaaaaaaaaaaggagattcgggtgaggatcagggtgccgggtggaaacatgggagcgagggggcagtgggatggtgagagggaaggtgctggaggctggctgagattccggcctccagcctcactattcaccgacacttaaggggcagccccgtctcccccttcgggctcatcaggagctggggcgtccacagccccatcctcactggccaccagtggctcctcctcccctttgaggctggggcctgacccagacttcagctcctccatcgccagggagccctggcgagacttccgtctgccaaagaaagtggtgagcgtgggccgacggctagacccctccccatcggggaacccagagcccttgtcgcccccggaccctcccacggtcactgtcacggccccctcctcagggacctgggctggcccagcccaggcgtccaccaccccgttacgcttgccgcctctgctcagcacgagggccccagtccgccgcttctgccgccggcgccacagcaggagcagagccacgaggactatgaccgccagcagggccacaagcacagccactggcagcatgcctcgtgagttctcatctgggttccggaagggcacagtgcttgcgttggtggaggtcgttggagacatcattgtagatagttttacgctagagacctggggtccactggccccgctggagggctccagagagccagttgtcatggtaacagggggtccagtggtcccagtggaggtctccagagagtcagttgccatggtaacagggggtccagaggtgcctttggaagtctccagagagacagttgccatggtaagagggggtccagaggtgcctctggaggtctccagagagctagctgccgtggtaacaggggctccactggtcctactggaggtttctggagagttcgttgttatggttccacctgtcacggtgtgggatcctagagagtttgctgttatgggaacagcaggatgactggttgcatgaggggtttcctggggcactgatgacatcttgatggaaacttcctggtaggttgttggctcaggtaaaggggaaccagtgctggcaccaatggaagtccaaagaggggatccctcattgatggaagttgagggaggtagggctgaggtctggtccccagtgctgtcggccttagggtcacttgttattgaagtggtgtacatctttgagctcaggggctcgctagtagagaccaaaggctctccggaggtgggtgtctgcactgctgttgtgctccccagagcgtctgggcttaccaccagcaccccaaggagaaggagaagcgtggccatttccaggcaaacaggcaggagcaagagctgggacctgagggaggcagggaagcgtgggatctggaatcaggattcctggctcttggctgaggaatgggatggaagtggtgatgctagggagggctgggctcagaggtgggtggtgggaatgt

SEQ ID NO: 15458 - RNA, 2523 nt, Homo sapiens
  source 1..2523: mol_type = other RNA
gctgggattacaggcatgagccactgcgctggctaggtcaacatttaatagttaaccattgctatttgttctatcaaggacatatcaaaactactagaagtttgctgccaccaccttgattcatgccacagtgccaacagttgacctcacagatcctccctgaaagggtcttgggactcccaggatctgcaggccgcattcttcgagaaccactattctaggtacagccccactgtccttctaaaatctaaggtcacagcttaaacttcagggaaggctgtagttttggaggccattgtcacattagaacccatttagaagtgactgtcaagagacaacttgagtgagtctgaaactgcctgctgatggcagtgtttctcaactggtttaaatcgccagtcccctaggaagccttcttcctgatcactccctgccatgaaaatggaatatcacagacacactatatgtgctgtgggccttaggagggccacaaacaactgcttgtgatttttttttatccttactgaagaaccaatttgcatccctgttgagaatacagggcttgtggccagtaataactctcccttttaggattcctgtctttccccattttttttctatccccagttgccatcacagcgtaacggtgcagggaggtatatgagggttgctaagggaaagcagaggtgcccctcactcaaacctacattcagaaaaaaatttccttcattattgattggatgtcttaaatgcaaagacttacacagaaactgggaagggaggacctatttcagacaaggattcaccatggaatttttatgaatatccttataaaataggacttgggatgcagatggattatttctttaagtcttgcaacttcagaaaagcctgagacacataccccctcctactatatatagtgattataaatagtatatttacctccaaaaaatttaacactgtgccctaatgcaagaaaaatctgtggtataacaatgtactcatgttctgtagctctttactgaaggcctcatgtcaaaggcggggaaggaaagcaattctgtggctctgcacttctacccaagtctgaagagaagtgagccaagttaaatgaaggtcaaggatgctcctcctggtcctctcaggggctggtaaagtcttatatgacgttttctggggagtcattactctgtccaaagtcgaggtagctcagaggccttcaggccgctgatacttccagaaggccacctccccatcatcactgcaggaggccagtagccctggctccttggggttccaggccacacagttgacatcctgggaatgggcctgatgcaagtgggctgtcagggagaaggtgggctgctgtggatccgagttgggatcctcctgaaacacgcggatcgcgtcatccccacaagctgtggccagagcccctgtcagctgacaccaagcaatgtcataaatggtccttgagtggaagccggacaaagtacagatacatttccaactggggtcagagccgctgcatgccaccccttgttcattgcctggtagatactgacgccagatacgcacagtacggtcatcactacaagacgccaggcgctggccactcgggtcaaaggccaagctccacacagtggattcatggccctcaagggtggcacagcatacccagtcatcctcttcctcccggtacagcttcactgtgtcatcatagctggcagaagctaagagctcctgacttgggtgccaaaccacatgcttgacatcctgtgtgtgggagttgagaacactgacacattcatactcatcctcttcatcaactgtgggagagaaaaaggggacccaagagccgaccctgtcagggacacagagggggctgtcaggtggttcccaatccacctggagggacctggcctcaccttcccagacccaaacgctcttatctcggctgcaagtggccaggaggttgccagatggggcccaagccactgacttgacctcattttcatggccctcgagagtggttacacactcaaagtcatcctggttcttcttccaaatgcaagtggtagcatcaaagctggcagaggccaggtaattaccgcagggggaccaggctaccttccgcacggtgcgctggtggccttcagaaaggacagacttgcagatccagctgtcaccctccgtgccccagatgcggattctccggtcgccgccgcacgaggccagcagggtccccgcggggttccaggccaggaaccagcagcgggagtccgggtgcgccgggacacggcccagcagcaccagcgagtccttcatgtcggcccgacgcagggggaggtgggggcgggcagagtccgctgagcagacagcgggtctcaccgcgcgcgtctgcgtaccgcccactccaggcttccgcggccgacagaggctcccgcttccgccggaggacctgggtcgccccggaaactcaactgcccactgctgcggccgccataccctctgggagtt

SEQ ID NO: 15459 - RNA, 2358 nt, Homo sapiens
  source 1..2358: mol_type = other RNA
gctgggattacaggcatgagccactgcgctggctaggtcaacatttaatagttaaccattgctatttgttctatcaaggacatatcaaaactactagaagtttgctgccaccaccttgattcatgccacagtgccaacagttgacctcacagatcctccctgaaagggtcttgggactcccaggatctgcaggccgcattcttcgagaaccactattctaggtacagccccactgtccttctaaaatctaaggtcacagcttaaacttcagggaaggctgtagttttggaggccattgtcacattagaacccatttagaagtgactgtcaagagacaacttgagtgagtctgaaactgcctgctgatggcagtgtttctcaactggtttaaatcgccagtcccctaggaagccttcttcctgatcactccctgccatgaaaatggaatatcacagacacactatatgtgctgtgggccttaggagggccacaaacaactgcttgtgatttttttttatccttactgaagaaccaatttgcatccctgttgagaatacagggcttgtggccagtaataactctcccttttaggattcctgtctttccccattttttttctatccccagttgccatcacagcgtaacggtgcagggaggtatatgagggttgctaagggaaagcagaggtgcccctcactcaaacctacattcagaaaaaaatttccttcattattgattggatgtcttaaatgcaaagacttacacagaaactgggaagggaggacctatttcagacaaggattcaccatggaatttttatgaatatccttataaaataggacttgggatgcagatggattatttctttaagtcttgcaacttcagaaaagcctgagacacataccccctcctactatatatagtgattataaatagtatatttacctccaaaaaatttaacactgtgccctaatgcaagaaaaatctgtggtataacaatgtactcatgttctgtagctctttactgaaggcctcatgtcaaaggcggggaaggaaagcaattctgtggctctgcacttctacccaagtctgaagagaagtgagccaagttaaatgaaggtcaaggatgctcctcctggtcctctcaggggctggtaaagtcttatatgacgttttctggggagtcattactctgtccaaagtcgaggtagctcagaggccttcaggccgctgatacttccagaaggccacctccccatcatcactgcaggaggccagtagccctggctccttggggttccaggccacacagttgacatcctgggaatgggcctgatgcaagtgggctgtcagggagaaggtgggctgctgtggatccgagttgggatcctcctgaaacacgcggatcgcgtcatccccacaagctgtggccagagcccctgtcagctgacaccaagcaatgtcataaatggtccttgagtggaagccggacaaagtacagatacatttccaactggggtcagagccgctgcatgccaccccttgttcattgcctggtagatactgacgccagatacgcacagtacggtcatcactacaagacgccaggcgctggccactcgggtcaaaggccaagctccacacagtggattcatggccctcaagggtggcacagcatacccagtcatcctcttcctcccggtacagcttcactgtgtcatcatagctggcagaagctaagagctcctgacttgggtgccaaaccacatgcttgacatcctgtgtgtgggagttgagaacactgacacattcatactcatcctcttcatcaacttcccagacccaaacgctcttatctcggctgcaagtggccaggaggttgccagatggggcccaagccactgacttgacctcattttcatggccctcgagagtggttacacactcaaagtcatcctggttcttcttccaaatgcaagtggtagcatcaaagctggcagaggccaggtaattaccgcagggggaccaggctaccttccgcacggtgcgctggtggccttcagaaaggacagacttgcagatccagctgtcaccctccgtgccccagatgcggattctccggtcgccgccgcacgaggccagcagggtccccgcggggttccaggccaggaaccagcagcgggagtccgggtgcgccgggacacggcccagcagcaccagcgagtccttcatgtcggcccgacgcagggggaggtgggggcgggcagagtccgctgagcagacagcgggtctcaccgcgcgcgtctgcgtaccgcccactccaggcttccgcggccgacagaggctcccgcttccgcc

SEQ ID NO: 15460 - RNA, 4616 nt, Homo sapiens
  source 1..4616: mol_type = other RNA
gctgggattacaggcatgagccactgcgtccagcccatattctatttatatttctgtataatttttattatgaccataaaaatcaccctgtagtcaattacaatttaattggacatttaaaagtaactaaaagtgtataattacactgtttggattagaaaggataaatgctagaggtgacagataccttatttaccctaatgtaattactacatattgtatgcctgaatcaaaatattctctataagacatatatacacatactatatactcacagatagtaataataaattaagaaaaaagattaaaaatttaactaacgggaacaatattcttcatttgcagtttactggcaaagtgattactagtgatgacattccactacataccaaatagtatacttcttccatcttttgcttacaccatttgagtaaggccggataggttaaagttagtggcataataatgcttcattaaatgcacaatagttttaagatggtaaaaaataaaataaaattaggctggacatattggctcacacctataatcccaacactttgagagcctgaggtgggtggatcgcttgagctcaggagtttgagactagcctgaccaatatggggaaaccccatgtctattaaaaatataaaaattagccaggcgtggtgtcacgcacctgtagtccccactactcgggaggctgaggcaggagaatttcttgaacttgggaggtggaggttgcagtcattgtgctgagactgcactgctgccctccagcctgggtgacagagcaagactccatctcaaaagaaaagttaagtaagtaaataaaatataagttaagttcacacatcatctaacaatttttaaatatattgcattttattacgtaacagtaaaattagtaaaataattgatatactttaatttataatttctttctctcagtataatgtagaaaagtattactctgaacacctaccttaaacattacttaatataggttaactacaatgagcctctccacttatattttcgtcatgcatcttacattttaatgtccttactgttttatagaaaaggtcataaagaatgcccaactcataaagaatctctaatatctctgatgcagcaacaattgatcacatactttcacgtgaatataataaagtaacagcataatttgaaagctgtattacatcattcacttttcaaaaaaattgttttcaaggaaacaaatatactttcaatgtaaatacaaagcttcaaaaaatctccttttaaagttatatactaatttatacaaacttatatacaaatttaacaactttagttgtgaattcatttatatactcaacactcttatttaatgtaatgtctgaagtgtcagtgccttagttattctgtaaattctgatatttacatacaattaattttgaattaaatattttttcatgtttactgcatctgcaaaaatatattttagtataaactctgctgttttctaagctgtagttttttttttttaaagtgtttccaaattcattacatttgcaggacccttctccaatataagttctctgatgttgagcaaagcttgagcaactgcttcaggattttcctctagtacaaaatgtgtgtaataaacctcctgtatatttgtaatggttgtcttcagaataaatactcttcttcactttaaaggcttatattttctgaaagattttttgacagtaattgcacttttaatgctttcattaactatgaaccttcttatgttgagtaagatgtgagtaggcattaatgggttttccatattctttatatttgtacaatttttctcaaggataatagctttcctgcaaaataagatgtacacattgattaaaggttttgccacattcttcatgcttgtaggaattttgccagtatgaattatcttactatcaaatgtggcaaccatataaaggctgtttcacattttatatatttctagggtttcacactagtataaattttttatgtatagaaaggatggaagtgttgaaaaaagcactgtcacatctttcaggtttgtagagttcctcttcagaatgaattatcaccatgtctcttaatagtaagaacttgtggccaggcatggtggctcatgcctgtaattgcaacactttaggaggctgaggtgggtggatcatgtgaggtcaggggttggataccagcctgacaaacatggtgtaaccttgtctctactaaaaatacaaaagttagctgggcatgggggtgggcacctgtaatcccccttacttgggaggttgaggcaggagaatggattgaacccagaaggcggaggttgcagtgagccgagactgtgctattgcacaccagactgggtgacaagagttgaaactccatctcaaaaaaaaaaaaaaaaagacagaacttgttatatgctttgccacattcttcacacttgtagggtttctttccagtatgaattatgtgtaataaaggttgagaagttccttaaaaaatctgtcacattctttatatttgtagagtttatatttcatatcaattcttagttagaaattgagggctggttaaaagattttccccattcatcacattcacatggtttctctccagtatgaattatcttatgtgcagtaaggtgtgaggataggtgaaaagctttaccacattattcacatctgtagggtttctctccagtatgaaatctcttatgtgtagtaagtttagaggagtgcttaaaggctttgccacattcttcacatctgtagggtttttttccagtatgaattttcttatgtgtagtaaggttagagaaatgcttaaaagctttgtcacattcttcacatttgtagaatttctctccagtatgaattatcttatgtgtagtaaggtgtgaggaccgcttgaaggctttgccacattcttcacatttgtagaatttctctccagtatgattctctcatgtgtagtaaggattgaggactggttgaaggctttgccacattcttcacatttgtagggtctctctccagtatgaattttcttatgtgtagtaaggttagaggagcacttaaaagctttgccacattcttcacatttgtagaatttctctccagtatgaattctcctatgtgtagtaaggattgaggactggttgaaggctttgccacattcttcacatttgtagggtctctctccagtatgaattttcttatgtgtagtaaggttagaggagtacttaaaagctttgccacattcttcacatttgtagggtttctctccagtatgaattatcttatgcgtagtaaggtctgaagaccgcttgaaggctttgccacattcttcacatttgtagggtttctctccagtatgaattctcttatgtgtagtaagggtagaggagtacttaaaggctttgccacattcttcacatttgtagggtttgtcttcagtatgaattcttttatgtgtagtaagggtataggagtacttaaaggctttgtcacattcttcacatttgtagggtttttctccagtatgaattatcttatgtgtagtaagggttgaggaccggttgaaggctttgccacattcttcacatttgtagggtttcttttccgtatgaattatctcatgtttactaagggttgaggatgacataaaggctttgccacatttatcacacttgtagggtttctctccagtatgatttctcttatgtgtagtaagagtggaggagtgcttaaaggctttgccacattcttcacatttgtagggtttctctccagtatgaattttcttatgtctagtaaggctacaagagtggttaaaggctttgccacattcttcacatttgtagggtttccctccagtatgaattttcttatgtgtagtaagagttgagaactgcttaaaagctttgccacattctatatatttgaaaggttttttcccagtatgtcctctcttttgtccgtttgaatttggaaattgatgaaggactttcacatatttatcacattgacatatttttcttggggtagttgtcaaacattggttaagttcattataaccttctttgtgcaccttacactcatccacacttatacatcctttttttaactgtaaattgtcatgttcacatttttcatatcttctcagtaccactttttggaaagaatctttcatgctctgctctggccaaaggtcttgggcaaaatgagaacacattactgagggtttggctatcatctcatttctcttcatggtcaaaggttttcttccttgctccagacaggtgatcaggtctggcttagaaacagtaataccaaggaagaccaggttactgtagttctctaacatcacattcctatataaattccgctgtgcagtgtccaggcaatgccactcctccagagagaattctatggccacatctctaaattgcaatggtcccatttttggcttccaggaggtcccggtgtcttagctgtggatctcccaatacctgcaggacacggggccacacagcctgggcctttaggagaagaaccagacctggagctctgactgcagcgagagac

SEQ ID NO: 15461 - RNA, 1956 nt, Homo sapiens
  source 1..1956: mol_type = other RNA
gctgggattacaggcatgagccactgcgtccggccagatcttcttatttatattgggctaagcatcatatctggcaaaatgaaagcaagtctttgttatatgttcagtttgctactgtcttccatctcctggttcctttgactctatgtcttcatccttttccaagaagtctcttgcacatcttccttcccacaccacaaaagcatctcttgcacgtttgggagtttgtgttgtccaggcggatgctgtaggttcaacttcagccaataaaacttcctctcacctgaggctataggtgtctctgggatcagtaagtcacttactgagcctactttcttaccccagattctgtgcaccaaatcggagaacaataggctggttgtgcaaatagacaatgccaaattggctgcagatgacttcaggaccaagtgagttggggttggacagggatgggaaggagccaagtgagagttggggttggatggggatgggacaatgccaagttggctgcttctgtctcatgtggcatcggatgtcattgacccagaccccaacccagtagttatagcagaagagaacaaagggcattaagctcaagatcctgaaaaactatccgctctccagtggtttagcattaacagtttacaacatgtgctagaatgcatcatccacctggtaagcaacttgtgaagcaggcgggcagggatagaatctcctccacaggtggggaccctgaggcttggggtgctggtgtgacttgccagaagccatgtgggtaccgagtggcagagctgggacttggccttaaattttgtaccaaattttcctttcttgaagcaatttcctgtgaaactgttgccttaataaggatatgtttctgtgctgcagcttgattaatttgtgagtgctgataattcatagcagaaatcatgctccatagcctaagatgaaaacatgtgaaagtcaaagggttgacaccacctgaggagggtctaccctgggtgctggaagggcattgtgttttatcatctttcttcggggcactgtgcaagtctcactcttctagagctaaagaaagccatttccttcctctcatgctggcaatgtggcttttactctaatagggaatccagggtccctttgggtatggggcttgtagagaggggcctgcagtgattgcactgtgttgcaaatgcctggttactttgccacctcccttttgggccattgtgtgtaaaggcaggtgctggctgtgtgtccatcacagtatcctcagtaccagctgctccccttggttcatctcaggtgcttagtattgactgagtggggaacatcctgttgctttctgggctttgagcacactacacaggataagccaactcacaattagatggcaaagggcaggccagtggacttacagctgcgagctgggagtcatgtcctggtgccccttcctgccctctaactgtcactcctgcactttccctgttacaggtacgagagagagcgctcgctgcaacagctggtggaggctgacatctgtggcctgcgcagggtgctagacaacctcaccctcgccaagtgtgacctggaggcccagctggagtccctgaaggaggagctgctttgcctcaagaagaaccatgagcaggtgtgtgacccttggtgtgatgcattgagactttctggaggtgaattcaggctcatctggggggaaaaaacggaggcttccttctgcttgggattgaagctttgcaggtgagctctggcttttggtgggagattgcttctcatccacagcttctggaagctgctaggctggtgcaggcagcggtttatcttcagaggagcacagggaaattacttgatgcccatggatcctgtggggatgccacagggctgaagcgatgggccatcaccaccgcctctcctgtggtctccaaagcaacaagaacc

SEQ ID NO: 15462 - RNA, 332 nt, Homo sapiens
  source 1..332: mol_type = other RNA
gctgggattacaggcatgagccactgcgtcctgaccttacaagcttccaccagtctgcagaagaatttctttgtctgacattttgagagaaagtagtgtggccccaagctttttttcctgtttagtccactgttcacatgctgaaatatttctgttcttgtttttatgctctcttgatttgtagtacttcaccttcctccacatcatcacatagctaaatctttctcacacttaagaccagttcatcctgcaggcctcttgactggtgaagtcagccagccatctcagcagggaagaacaaccttctcaaccaaaactgcaatcaggaaagc

SEQ ID NO: 15463 - RNA, 2248 nt, Homo sapiens
  source 1..2248: mol_type = other RNA
gctgggattacaggcatgagccactgcgtctggcccagtcttcccctattctctggaccacagtttgaaaatcacagacaggtcaacctagatccttccagctctagttttctactgtgttctttcctcttgagaagttacagctcatcatgggcccttaataacagaattcaacagaaggcatcatctgaaaacaaagtcaattcagaaactgttgttgcaagaaggcaaacagaaaaacggcaccatgtcccactggaatctctttcagcgatggagagttttgttttctggtaaaaaatatagaaatagtggttgtccttgaggggacttgtggtttggttctaaacctccccatggagccgagtggtgtccctgagggtgaggagggcagaggtctctgctcagagctgctctgagcccatccgcaagtttttgatctccagttccaactgtttggcctggacctctcgctgggtcaacagctcccggagccttcggatctcctcctgttgccggtagaacatctgcagcaactcattctctgtctttggtggggggcattcgaaaacgtcaaagccatttgtcagccaggttttcttctcctccagcctgtgttctgctgcccaccttggcatcttctcctccaacagggaggaagacctccagccatcttctgcagccagcttttctgtctgattcaagagccggggtgaggctggggccatggaattgaagataggtctctctgcaggcagtgggtggggtctcagcagctcagagccaggcctaagggacaccaggattgggtctcgattcatcccgctgagccactcctgggccgtcagggagggctgggcccctgctgttggagggtatatgtcctcttggtaggattctgaccgccggggcacaatcatggagatgggctcgatgaggcttttggttgtgatcagcttgtagaagcggaagatctcgcaggaggacacgtcgagtcctctctttggcatgacaccgatccccttctgtgggttataggagcggtactcagtcaggtagctcaggtgaggcttgtcggcgctcacctcgtagtagcggatgttgccatctcccttccccaccacgtagagcatgctggtgtccgcgtcatagaagggaaacagcacgcccgaggagccgtccaggtcctcctccatcagaggcacagagaggttatcctggtcccacaaggccacctgccggttgttccatcgggatgtgcctgtggacatcagcttcttcaggttccccagaaacagcactttgctggcccggtgccctttgtagctggcctcctggaggacggtccctgctcgggggtcaataacccgaatcttgcggtctttgcaggtggtggccaacaggctgccgttggtgttgaaggacatggagaggatcacatcttggtgacagctaatcgtactcatggggcttgtgatgacagactcctttgtatccaggttccagatcatcaccttgtagtcatagccagcactgaagaggatgttggcggccgtggggtgccactccaccaggcctactctgcgcgcgtggcccacgagttccttcctgtaggccgtgaggttcctggtcagcagctgcttggggatgctccagatcttaattgtggcatcttcagaacaggaggcgatctcaaaatcatcaaaagggttccacttgacatccaaaacgttgcctctgtgcccgcagacttttgggtagtgggggtccaacttccctgtctggtgcagggggatgacgaggaaggcccctccaccagcacactcagtcacaactgcaatgaagtgggggttcacggcacagaagtggttgtcgtgaacgctgcgggtgataggcacggagtcgtagcagttctccttgctggctggtttgccaaagacatgacggaacttggagctccggtactgggggtgccatgacatctgcttgttaacatggagataaatgcctctgctcacccttaatcagttccccaggcagagtctgcaacagctggcaggagaggatggtgaggtacctcctctctgcttccagcctccaggagctccacctaaattgtttgtccaggctgggcctgcaggccagaaaggcaggaggccagactgattgcccttctcaaatttcaagtgccagcagcctgggtttatgaggattaaaagagtccagcaaagatgtcagtgcccctgtg

SEQ ID NO: 15464 - RNA, 2061 nt, Homo sapiens
  source 1..2061: mol_type = other RNA
gctgggattacaggcatgagccactgcgtctggcccagtcttcccctattctctggaccacagtttgaaaatcacagacaggtcaacctagatccttccagctctagttttctactgtgttctttcctcttgagaagttacagctcatcatgggcccttaataacagaattcaacagaaggcatcatctgaaaacaaagtcaattcagaaactgttgttgcaagaaggcaaacagaaaaacggcaccatgtcccactggaatctctttcagcgatggagagttttgttttctggtaaaaaatatagaaatagtggttgtccttgaggggacttgtggtttggttctaaacctccccatggagccgagtggtgtccctgagggtgaggagggcagaggtctctgctcagagctgctctgagcccatccgcaagtttttgatctccagttccaactgtttggcctggacctctcgctgggtcaacagctcccggagccttcggatctcctcctgttgccggtagaacatctgcagcaactcattctctgtctttggtggggggcattcgaaaacgtcaaagccatttgtcagccaggttttcttctcctccagcctgtgttctgctgcccaccttggcatcttctcctccaacagggaggaagacctccagccatcttctgcagccagcttttctgtctgattcaagagccggggtgaggctggggccatggaattgaagataggtctctctgcaggcagtgggtggggtctcagcagctcagagccaggcctaagggacaccaggattgggtctcgattcatcccgctgagccactcctgggccgtcagggagggctgggcccctgctgttggagggtatatgtcctcttggtaggattctgaccgccggggcacaatcatggagatgggctcgatgaggcttttggttgtgatcagcttgtagaagcggaagatctcgcaggaggacacgtcgagtcctctctttggcatgacaccgatccccttctgtgggttataggagcggtactcagtcaggtagctcaggtgaggcttgtcggcgctcacctcgtagtagcggatgttgccatctcccttccccaccacgtagagcatgctggtgtccgcgtcatagaagggaaacagcacgcccgaggagccgtccaggtcctcctccatcagaggcacagagaggttatcctggtcccacaaggccacctgccggttgttccatcgggatgtgcctgtggacatcagcttcttcaggttccccagaaacagcactttgctggcccggtgccctttgtagctggcctcctggaggacggtccctgctcgggggtcaataacccgaatcttgcggtctttgcaggtggtggccaacaggctgccgttggtgttgaaggacatggagaggatcacatcttggtgacagctaatcgtactcatggggcttgtgatgacagactcctttgtatccaggttccagatcatcaccttgtagtcatagccagcactgaagaggatgttggcggccgtggggtgccactccaccaggcctactctgcgcgcgtggcccacgagttccttcctgtaggccgtgaggttcctggtcagcagctgcttggggatgctccagatcttaattgtggcatcttcagaacaggaggcgatctcaaaatcatcaaaagggttccacttgacatccaaaacgttgcctctgtgcccgcagacttttgggtagtgggggtccaacttccctgtctggtgcagggggatgacgaggaaggcccctccaccagcacactcagtcacaactgcaatgaagtgggggttcacggcacagaagtggttgtcgtgaacgctgcgggtgataggcacggagtcgtagcagttctccttgctggctggtttgccaaagacatgacggaacttggagctccggtactgggggtgccatgacatcttgatgactgccgcgcaggtggcggtggcggcggcggcgtccagctccggctccgcgctcctcgccgcccgccgactc

SEQ ID NO: 15465 - RNA, 1144 nt, Homo sapiens
  source 1..1144: mol_type = other RNA
gctgggattacaggcatgagccactgcgttcttgcttttcttcaaaatccctttgtcaaagtctttggtttagtacagtttttaaacatatccttttcatatttttcattcaccactgcatcctttttttcataaggtcccaatttttttgcaacacaacttatggttaggccaggatgtgctcctttgattgtgagggggtactcagaacaaaacaaggacgacacttgggtggggtaccatgagcagcagcttggccttggcctttcttcgggaacttgttagaaatacgggaccctgggtcccatcctagacccagtgtatcccactctgcttttgaacaacactctctaagatgcctatgcataaatttgagaagtaccactttagcatgttgtagaaaattgagacagcttgactgaagcttcaggatgctttgtcttgtgttctttccagcagtttgcacaagatgccatgtagtgccatttggcctcttggcctctatggatctgtcttgcccatctttaattatttttccttaatgaggctctgggtggggcgtctgtgtggctctcagttggcccaatgcttgctgtgtggaatccagcattgtgctagcagggggcagaggcagcatcaaaacttaattctaagttctgcaagcctagagggtttgagaactgtttatgatgaaaatggctactggattgtcaataaactatatatttttcccccattttgctacagtcttgtgattcgtggtgataaagacgagcaagctgtgctgtgcagtaaagacaaaacatacgacttgaagatagcagacacttccaatatgttgcttttcattcctggttgtaaaactccggaccagttgaagaaggaagattcacactgtaacattattcacactgaggtgctcttttctgtactctgatttataaaagtctggctcttcgcaaactttgtcctccattcttctcaatatgcttgtactagaaaactaccttccctccttttcttcctgctgttctcgcttcatccattaaatagttttttccctatcctaaattttaacaattctttacgataagacacatgcgaagatcgcaagccctgcccattgacaagacttcctggttct

SEQ ID NO: 15466 - RNA, 1380 nt, Homo sapiens
  source 1..1380: mol_type = other RNA
gctgggattacaggcatgagccactgctcccagactttagtttttgtttgtttgtttgttttgagacagagtctccctctgtcacccaggctggagtgcaatggcacgatgtcggctcactgcaacctctacctcctgggttcaagcgattctactgcctcagcctcctgagcagctgggattacaggcacctgccaccatgcttggctaatttttggtatttttagtggagatggggtttcaccatgttggtcaggctggtcttgaactcctgactttgtgatccacccacctcggcctcccaaagtgctgggattacaggcgtgagccactgcccccggccctggcttttaatattttaaatctcagttttctctgacttttagatggcactcataagtagcgttcccgtctatgaacaggacacaatcaacaaaaacaggtgctggggagggccgtgtttcatgggcagtatcgcaaaaaagcagaagaaattcctttccactacgtaggagcccacagaaatgtatgcactaaaatatatgcaagcaaaagcaaacaaaccaaaagctgcattcacagcgtagaccctgcaagagcaggaacactccctgccccagatacatacaccaaacacaaatacacatcaaagatgctctctcaggctcatgaatgtgcaggcacaggcaagcacacacatgcccgaacaaaaacacacaaagaacaaggatgaacacacacccaagctgtggctgccgtgcgtgtctatttattgttgctgccaccctggaggagccccagtttcttctgtagctttcttttctgggggatcttcctggctctgcccctccattcccagcctctcactccccatcttgcacttttgctagggttggaggcgctttcctggtagcccctcagagactcagtcagcgggaataagtcctaggggtggggggtgtggcaagccggcctggatcctgtcctgggtcctccttcctccgcagtcccgtctctattgctgggtgtagtgtccatggtctggcctcatctccagctctgtctcagcgccgtgcccctcgcttcttcctctctgaattctgcagcttggtcaccagtttcctctcgtgcccgccagggctggggcggttggtgttggcagcagcttctctcttggtgcgacctttccggcctccacctccgaggtaggaatgggccaggctatagaggtcagattcatccaggctggagtcctcgtcctccgggcctgggggctgctggggggcgctggttgctggtgggaaggtggccatcgtgcctggcttgtcttccctgcctctcttcttctcctaacgctttgtctgtctctgctttcctggc

SEQ ID NO: 15467 - RNA, 1434 nt, Homo sapiens
  source 1..1434: mol_type = other RNA
gctgggattacaggcatgagccactgctcccagactttagtttttgtttgtttgtttgttttgagacagagtctccctctgtcacccaggctggagtgcaatggcacgatgtcggctcactgcaacctctacctcctgggttcaagcgattctactgcctcagcctcctgagcagctgggattacaggcacctgccaccatgcttggctaatttttggtatttttagtggagatggggtttcaccatgttggtcaggctggtcttgaactcctgactttgtgatccacccacctcggcctcccaaagtgctgggattacaggcgtgagccactgcccccggccctggcttttaatattttaaatctcagttttctctgacttttagatggcactcataagtagcgttcccgtctatgaacaggacacaatcaacaaaaacaggtgctggggagggccgtgtttcatgggcagtatcgcaaaaaagcagaagaaattcctttccactacgtaggagcccacagaaatgtatgcactaaaatatatgcaagcaaaagcaaacaaaccaaaagctgcattcacagcgtagaccctgcaagagcaggaacactccctgccccagatacatacaccaaacacaaatacacatcaaagatgctctctcaggctcatgaatgtgcaggcacaggcaagcacacacatgcccgaacaaaaacacacaaagaacaaggatgaacacacacccaagctgtggctgccgtgcgtgtctatttattgttgctgccaccctggaggagccccagtttcttctgtagctttcttttctgggggatcttcctggctctgcccctccattcccagcctctcactccccatcttgcacttttgctagggttggaggcgctttcctggtagcccctcagagactcagtcagcgggaataagtcctaggggtggggggtgtggcaagccggcctggatcctgtcctgggtcctccttcctccgcagtcccgtctctattgctgggtgtagtgtccatggtctggcctcatctccagctctgtctcagcgccgtgcccctcgcttcttcctctctgaattctgcagcttggtcaccagtttcctctcgtgcccgccagggctggggcggttggtgttggcagcagcttctctcttggtgcgacctttccggcctccacctcctgtaaccaaggcaggagtcagaggtgaagtgggcataggcatgatgagaggcccgaggtaggaatgggccaggctatagaggtcagattcatccaggctggagtcctcgtcctccgggcctgggggctgctggggggcgctggttgctggtgggaaggtggccatcgtgcctggcttgtcttccctgcctctcttcttctcctaacgctttgtctgtctctgctttcctggc

SEQ ID NO: 15468 - RNA, 9657 nt, Homo sapiens
  source 1..9657: mol_type = other RNA
gctgggattacaggcatgagccactgctcccggccagaaaaccatattattttttaaaaaagaaaaccacccagtcaggcacagtggctcacgcctgtaatcccagcactttgggaggctgaggcaggcagatcacgaggtcaggagatcaagaccatcctggtcaacatggtgacacgccatctcttataaaatacaaaaaattagctgggcgtggtggcacacgcctgtagtgccagctactcgggaggctgaggcaggggaatcacttgaacctgggatacggaggttgcagtgagccaagatcgcgccactgcactccagcctggcgacagagtgagagtctgtcaaaaaaacaaaaaaaacaaacctgatgcatatttcctaaagactacaacattctgatattctatgtatagtatatatttttgcataactgaataaaacacataatttaaacactgttagtgaccaaagccaccatgtttgagaaaaggcaataaatttcagcaactgtttaaactgcttataaatatagtatgccaaagctggaagtttactggataggaagagtagcttagacagaaagcgtctctgaggctctatgactggctaggtacccgacccacgcgttctcagagtaccctgtgcttgtccctgttgtcacacccaacatgccgtgttataactgccagtctctgtgattacacactgcaggatccttgagggcagggatggtgctggttcactgaagtacccttcgtgcttgacatacagtaaagactccataaataattgtttgataactactgaatgagtaaccagccatcttcactcattgatctgctgggagcaacagaagcaggcaagagtagcaccacatgacacaggaataagaggcacggtttccaagagcaggccggacgcagtgactcacgcctgtaatcccagcactttgggaggcagaggcggattgcctgaggtcaggccgagatcagcctgaccaacatggtgaaaccctatctctactaaaaatacaaaaattagccgggcgtggtggcgggcgcctgtaatcccagctactcaggaggctgagacaggagaatcgcttcaatccaggaggcggaggttgtggtgagccgagattgcaccactgcactccagcctggcaacaagagtgaaactccatctttaaaaaaaaaaaaaaaaaaaaaaaggcacggttaccaagagcctgtgtttggtgtttgccagatggccaaaggctcccatcaaaatatgactgatggaatactcagacatgtccattcaataatgtccctacagtacgacatactatactcacctattatgagtgacaccaaaggatacatgatattttggctaggatcattttgactgttaagccaactcttacacacaccttaccaaaatttgcaaactgtctattaatcacaagcaactaagcaccaacaacactattcaagaaaggaaaaatgagttagggtgggttatattttactaggaaattcctctggctatattctataggaattaggtgtaatatctgttatgcaattgcttagcatagtgtttggcaaagtattaacaaagcctctttcccttctgcatgagaattttacctttgttaactttctagctctgttcccctggcaacctaataaaaattcatatgtcaactgctaggcaatgttacatatggtagacatgatgcccaattggtaaactgcatctggactgggagaactataaatgcctgataggaagcctcagctctgggcatccctaagtacagtgacgcttggaacaggcatgtcttttatagggacactggaggccatgtctatgaagctgttataagagatacttgttcctgtgggacaaggggctcttaagccggggaagcttccatacttgccccatgtagatctgtctccttgcacctgcactatgccacacagacagctgcagagactttcagagaagagcaactggttctgccttgctagtaagcagtgcttcccattctatatccttttaagtgaatctgatgccaagtgtggcagtttataaatttgaatgtttctaaaccttcagttgggcctaagacccttggagggcactgcagtattatttgcatgtttttctgatggcagtagatgctcctcaggggctatggatggtaaaagatgtgaaactgtttggtatgtttttctacttccaaaaaaatcctgaccatacccttcactgtatgcatgacagataatccatatccattacatgtcaccaagacctgtatatgaaattgatgccttccttcaaaatccccaagcttgttactactaaaccttcctcatcaaagcacataatccctgccctaacctccactgattaactgacaaaggtccagaaatcaaatgatggatataaaaattgccccccctaaaaccacaattgtcaatgaagaattggcagtagtaaaataatctacctggagggtcaagacggatgctaaatgttctccttcagttatgaagtttccatgtcatccgatcatgcagtcatgtgagttactgtcaccttttaaaactaggatatatttaggccgggcgcggtggctcacgcctgtaatcctagcactttgggaggccgaggcgggtggatcacaaggtcaggatattgagactatcctggctaacacggtgaaaccccgtctctactaaaaatacaaaaaattagctgggcatggtggcgggtgcctgtagtcccagctactcaggaggctgaggcaggagaatggcatgaacccaggaggcggagcttgcagtgagccgagattgtgccactgcactccagcctgggcaacagagcgagactccgtctcagaaaaaaaaagaaaagaaaaacaacaacaacaacaaaaactaggacatgtttaggaaccaaccaaactactctgaccccaaaacacttttcgtttttctctacagaaacatcatttgaagaaaagaattcaaatttccagcactacaatgaaaggtttgtggaacacagtactgttgagtggagagaactacaaaagcaacagaaatcaatgaaaacagtgcccatcatatgcacctgaataaagtgtccctttatcaggttagaagatagtgtgatcacatgaaaacacaaggcaagctacaagagaccagcaacaacaggaagcacagtgggaatgctcaaaacagagcataataggaacttctcacccatcccaaccctttgcccctccctaccccattacactagacttcacagagatcattctcttaatgcacaagggacacacacaagaaaaatctagagttccaaataaaacagtctgagttcagttaaccaaaggccactccactctttcctacggctcccagaatcagtgcatgcagccctacctgttgcctttctctccctggggtttgtcacgacatcaatgaacaataacaaaaaaaacccatctcagtattccaaaccaccagaatactcaattccataacatgttgcagaacactaggtcagcagcttccttaaggaatattcaaagtctggtggccaccaaaatatttacatcagaacggcatctttctgccaaatgatcagaatcatgatgcactatgtcatttcttaattattataggtaaggccctatttacattccttctcaacttttgagaagggggtcctcatcccccaagagaaataacttcccaagaatgccattttggaattccattacaagtaagagtcctgttcccattcatgcaatacatctaatatgagacgaaaatatccctttgtgaacttgggtggaatgtgccagaatagaaactaaaccactaacggtctgtgttgggctcaactgtaaatttacttagtataaaaataccaccaaccccacaaattaaacctcaaagacactgtgattataaatactgaccacctaaaggggaccaatttatgatctgatagtctagacagaggaagtatctcctttaaaagtgatagaactcagtgatccagttattgccagtgcctatacacaaactccaaatagtccaccagaaatgcaacaatctgagatattacgaaagaaagagaatcatttaaacattaggtgtcacattctgttttcttcccagtgattctgctactttaaaaattaacaaaatgatcagaacctagtaacgattctgggtgtatgaatgagtcagaattttctaagtttccacattataaacctaaatcagatcttgggcaagctatgaaccatctggcctcagcgcttcattttactaatccactattttctaaaatttgcgagagtataaggggctactaaatattatgaaggtcagccaggcacggtggctcacgcctgtaatcccagcactttgggaggctgaggcaggcggatcacttgaggtcaggagttcaagaccagcctggccaacatggtgaaaccccatttctactaaaaatacaaaaattggccaggcgtggtggcgcgtgcctataatcccaactactcaagaggctgagacagaagaatctcttgaacctgggaggtggaggttgcagtgagccgagatcacgccattgcactccagcctgggtgacaaagatgaaactccatctcaaaataaataaataaatacataaaataaaattaaaaataaataaatattatgcaggtaaaaggtagcttaaaatagaacacaaaattaagtccactcattaaagatcctttaaaaaatcctactttatcttacagcagagtttctcaacattggtattactgacattttgaattggagaattcattgttgtggggactgtcctgtgcatttcaggatgtttggcagcttccctggcctctacccactagatgccagtagccacctgcaaggcacgaaatcacccccaactgagaatcactgtcctacagtgaaatctctaatgtaaaatgttttacccagggatatgaagaggtcacggaatcactgaagaggatcatagctccactggagaaagcaggcaaagaggctgaactatgaggtagaaaagtcattaaaacatcagagataatttaaacagagaaagcaaaaatatcaaacactgttcctggccaagtaaatcttctacacatccatttaggtttcctttttgctgagatccctcttttaaaataacagcaaatatatgtatacatttttggagacagtttcgctcttgttgcccaggctggagtgcagtggtgtgatgtcggctcacagcaacctccgcctcctgggttcaagcgattctcctgcttcagcctcctgagtagctggaattacaggcatgcgccaccatgcctggctaattttgtatttttagtagagacggggtttctccatgttggccaggctggtcttgaactcccgacctcaggtgatccacctgccttggcctcccaaagtgttgggattacaggcgtgagccactgcgcctggccacagctagtatttttatttcagataagacaaatatctctggtccctgataattttcaatgagtaactcttgatctagaatatttttcttttatttatttattttattattatttttttgagacaaggtctcacactgttgcccaggctggagtggagtggcacgattccagctcactgcaaccttttccaggctcaagtgttcctctcgccacagcctcctgagtagctgggattacaggcacatgccaccactcctgactaatttttgtatttttgctagagacggggtttcgccatgttggtcaggctggtatcgaactcctgacctcaagtgttccatctgccttggcctcccaaagtgctgggattataggcgtgagccaccgcacacagccaagaatgatatttatcgaactacctgtgataagagaagttttaaattttccattctactgcagaccaatacgtggtcctgctgtacaggctggtatccaacctctgcaccatgtggccctctagctgaccagaactgaactggtccatacctcactcaagaagacaaagccatgagtcacagcaatgtcaaagtgttatcaacatttctatatgtgtattcttaatttctgactttccttgtagcagactggtagaaaacagtttacagaacagggcctctctgtgggccagagtttgagttgcactgttccagttttaactactattgagaagtacgacttaaacacctgtctaatgctttggctaacatttacaagccaatttataatgtttttgacttttttgttgttcaagaggtagaaataaaagtgacttttaccaccttttgaaagacaactacacttaaaggaagacaagaagatttcttttaaaatccattttggatattttaacataagacaaaattatggaaattgccttcaattacattccgaattcctaacactgcctgccctttagccctttaaagagttcagcctcttttgttacaataattgtgtggctggaaagtgggcgaaaggtagactgcttttaaaaacctgttctgctactaaccttccctttccctcatgaagatcttttaaaagatgaacattttagaaatgttacttggcattatgggcttatactttccctccaattaaagttctaggcaaggaggtagaaggcaggactcaactccaaaggccggactcggacatggaccaaattgaggactagctaaaacagggcggtggtgggagggtggtgcaggaagcagatttccataagaaacacttatcactgtgccatgtcaattaccattgccatggcaacacctggaagtcactgccccttatcatggcaaccacccagcggcttggaagttaccaccattttcctaaatattgctgcataatctgccccttaatttgcatgtaactaaaagtgggtataaatataagtgccgacctgcctctgagctactactctgggcacactgcctatggtgtagccctgctccacgaggagcggccccttagctgctgttgggcactgctgcttcaatacaagctgctgtctaacaccactggcttgcccttgaattctttcctgggtgaagccaagaactcctctgggctaagccccaatttttgggctcacctgccctacatcagcataaactaagtaaaagaatgccagaggcagctacatttccaagttacacagctccagcttttggaaattgctggaaaaagtaggggagcattttgagttttgcccaaatgagttgttttatgataacagaacaggttgtatgtgtagaatcgtcaaatgccaaaccagacagggaaaccatccagacctggggtcatagcctcccttctcagggctaacttaaaatttaattcaactgggcaagtcaggatgccataatgagcctttcagatcattcccatgttcgtctgcccataagtattccaagcctttaaaattgttctagatttagggagtaccttttatgatcatgtagccagaccgccctgcctgctttatatcaatgaaggtttctctttaatactttgccagaaaatttaatgtggaattcattaggaaaggcttggcaaaggtaaacttgatcccaaaacttaatggtttttagagaaagaggatgataacaaaggaatgcagaggactgaatcaatataaaaacaagcctggagattttcttatctttctcctaaccagagtttggacacacagcaagaaaaacaggagacctcagggcctgctttgactcactcagaattaaggagtggccagcaaagccctcagaaaccaagggcaccacacaaaaaggttatctgtcctttgagtcacaaaatccaacctctatcagatagtctaataaaaatgcacatataataacagtgaaaaaatgttcctctcagggttccacaaaattggacaaatggtatctttcaacaacagaacgagcactaacaagttttaaaacctcctcttccccaccaatttattgctacgtaagtgtctctcggtctgataagttaggctgaatttgtggtttgtcatcagaatcatctccagcagggtcattttcctcacccgactccacatagattggccagtcattgtctgtgtcgctcttttcttggctttcagatgaagcctccaccaagctaaggttgatgggcatcaaatcatcatcatcatcgggtgtgtctgtaacgcaggtgcagctgtcacacagcccgaagcgccgcagcccctgggacaggtgactcgtgaatgttctcctgcagcccttgcagatgattggacggttggatctgtggacactcagtgcgtggctccgcaggtgctcttgtcgagtgaacctcttgccgcaggtctcacaggggtagggccgctcgcctgtgtgtgaacggatgtgccgcttgaggatgcccttctgtttggcagtgtaagggcagaaaggacacttgtggagcttgatggggaccaccagcacatcacctgagtcctctccataccagtcagcctggacatccatcatggaactcatggctactcctgcaccttctggtcttccttccaaactcctagaaaagtgatggtctgcatcatccttgctcggggcagcgctgttgcgcaagagcgcctccaggaactgcttcacgtggtagttgctgtaagccaagtcaaccgcctggccgcttggcaaggcctcctccacgtgggccaggttcagcggggcagcatactgctgcagctgttcaccaacgtccacctccacttcatcagcatcaaattccaccttgggctctatccgtttgggtggagtagagaggttgctgtcagccgagccaccgccaaggctgtctctcaccaccagttccaaggggtggcagtctccgcagtcaccgcaaggggactctctcaggcactccacgctcttttctccctcggctggagaggagaccaagctcttggtaccacaggaggtcccctcccggcctgaactggggctttcactgtcaacctgatgagccgccgctgctgccgccgctgcagccgccgccgctgccgccgccactgctgcagccacagcagcctccttctccatctttcggcaaatgtcgagggatgacctaatgtatgtcttgcagaagttcaccacgtcattcatctgcaggtagctggcagccgacatcacttcaatcacattctccccacacaaatccaacttcccagaatagaggaaatctaagatgatggagaaggcatcagaggtgacaatgtccaaggaggcggtgctatgccgcccgctgtcctggatatagtgaatgagcagggctcggaagtagccgctgttagcaaacaaaatgttcctgtgggccttgaagatccgcccttccacaatgatgctgcagtcacagaaaaagtccctctttctctgttcattcagctcccccaaaagcttggcataataggattgcatctccattgctccgccagctgctgctgctccagagcaaacctgtatctcttccagcgggttccagcagcgcagccacggagc

SEQ ID NO: 15469 - RNA, 730 nt, Homo sapiens
  source 1..730: mol_type = other RNA
gctgggattacaggcatgagccactgctcccggcctaataaatacctgttgttttggtgatggcagccctaagaaatgaagacagagagcttaggcaaatgtccacgatcacacagcctgtgatgacagaggagacgggcgcgtgtaggccctgccatccccattccagagctctgtcctttgtccagggctttcttcctctgaggcttcatgcatcagttgtctgtgttgtctgtgtaagttttctccatcttttatttttgttctggatttctaaaataatttccttcaaatagacttttcttgtcttctgacccctgctgcatacaactttttatttggaaaaatttaaaaccttggcctcccaaagtgctgggattataagcgtgaggcaccatgcccggccaaatttttaaaggcataaagactatgtcttacgcttttctccatttgcagaacacagcaaaaaccttcaagtggaaatggaatttccagatgcagaatagaataagtgccatcaaaaggtagggtaattgccagctgcaactgagatcctcagtgttcatttatccaggtcatttattcgtgagtcatggatttgtggaatgaaaactgaacactgagccagcagttccctgaaactaggaaaacaataagttcttatttccctgacaaaatctggctacagttcagcaatgcagtaaaaaatccttatggattttctcattac

SEQ ID NO: 15470 - RNA, 1028 nt, Homo sapiens
  source 1..1028: mol_type = other RNA
gctgggattacaggcatgagccactggcccaaatcctgagtttcttctcgtcttttttatagtgcattgatccaaatcaggcaagtgtatgtgaccccacccctgccctgatttaatgtttacttccttttcttcatagttttataacttgttgccagtgaaaggatcagaatttgggggtctttcgtgtttgaggaaacgcagcccaggaagggaacccaacacgttttacctggcagcgtgtggctgagcctggagtgtcatcttgggcccctgactctgaggtgaaggctgtttctgcaacatttgggtctaacctcgtccttttactgcgacctgcctcaggaccaccttgcatttgtctctcttcagtttcctcttttttggtactatatgcgtacaacttcgagaagcttctgtaattttagttcagtttgtgtgttgtgcagccataccattaactgagcaggttcttttcctcaccgtctggtctgaatttccttgtcctgcggaaaggcattgcctgccacgccttgttgagttctctcatctccgatcacaaggtccaataggttgtctgcaagctgaggagcaaggaaaccagtccgagtcccaaagctgaagaacttgggagtcctgctacagtactgctgtggtcccccaggacagattcttcaacttctttgcttccttgtggcatcagcttgaggaggccctgcctcaggcgggtaaatctggagaagtctgggtcatgggctagcaccccagctgttagtggggctaggtaaaactagtatctggccctttccgaatccaggagggatgaccatgggaaatgtaccaatgcagtaaaggaagatgctgaacagctacagtgatcacaaatgtcagtgaaggaagcattaatctgtgggtgataggcaaacccactggataggtacaataggctagagtgagaaaagagtagaggaagagctttggaaatgacagcatggaagagataggcagaggaagaggagttagaaagg

SEQ ID NO: 15471 - RNA, 7801 nt, Homo sapiens
  source 1..7801: mol_type = other RNA
gctgggattacaggcatgagccactgggcccagcctaaatagtatatatttttaaatatcctttcagaaaaggccgcttatccagaaccattctgaagacagtaaagaactgctgaagaggaagaaaaaactggctgtgcaatagtcagacctcctctgaacaaagcctcctggagagaaacagctgcagtggaggcattactcacccatgttcagaggcaacggaaacgatttagaatcacaagcttgtcaagtattggagctggaagggaccttagggagcattgaatctactcacttcattttacagatgaaatgaagacaagatagatggagagtcttgcccaaagtcacatagagctggcatccaaatcactattgtttctcaaaaatatcacatggtggcaaatggagcataactctgtggggctggacgacagctaaattcaagcaacatttgttcattaagcacctactatgtacaaggcaccttacaagatggtactgaagatacaaagatggatgagacacagtcctgcctccaagggcttatgaaagtcattggaggccatgcttcaaaacctttcttagcagaaatattactgaccagggctaaggttgctggtgataacaaggcagctgctgccctggagaggtgatctcacaacaggtggcactttctccccttcactatctatcagaactaatgcctgttactcagctgctaggcattaaaattcttgaaaccctaaggacactcttctctcctaggcctccagtcaaacctgaagtcttagcctctcccacccacagcaatgacaggagggcagtagcgctccagaccctcccctcaattcttagtcaactgttcgctttctcccttgtgcccagcctaggccctctgcaaggactgacaatttcccaaggtactgtcaaagtgacccaggaaaatgtcctaccatatacatcgctggtatctaacttccactgccccatcaaccacctctcccacctctacatgggagctgaaataactccagtccctgatgacacacccaagcctcaattacccatactccaaaagatgagaaagatgtaatggttggttagaataaagccgattcaagaggcagtggaaaacagtgatttgataataaaactgatctctcacatttgtacggcgctttccagtttatatagtgtttttatccagttatctgattatattcttaccacaactctgtgaggtagttagtgaagtattattcccattttatagctgaagaaccttaggcttgagagaccaagcggtttgcccaaagttacccagctaaggaagtgtggagccaagtgtccaggtttcttgactccaaatccagtgctcttccccctatatagtctataattggcaggcaattgaatgaattgcccatgatcatatacctgctaagtgttggtgatgggattaggtttcagtctccaaatctgttagtacggtgccccttcaccataccaactaactgggccaatgtgctcagaatgtctaccatggaagagatcagaagaacatctagttagttaactactcttttctatgtctaggtcatcagttctctccttcatcctcccccaagtcaacaatgtatcccaactggcaaagcctctaaaacatgcactattcctagaacagaacccagagtcaggttacaaatttaaacttgcaactcctcttccattggtctactgattattcagtcattgctattacagacagatgggaaagagataagctgagcaaatctcagttctgccattaaacaaatgtaaacctttaatttccatcatccttccccacctcggtcagcaatttgacttcttaactcctgaactacaaagtaaaatccaatctgatctagggttagggagcaataaagcagtgaataatatccctgaagttcttggcgcttttctctggctagtatattacaacaggaggccctatcgtctgattttcatccagtgggctcagctggatgcttccaagcactctcacacctttcctttgtgtgcatctcagtactttagctttaggattggttgagtagcagggatatttgagatgaaagcaataagaggaggtaaagggaagctgcaagtggaaggcagagctaggacctttcctcttagttctctgctcgttaaaatgaaaacagctattattgcatcattagtggaagaggggaaggaagcttcaggatcatgacttaaaacctgactccagaaacacttctactgaatacaggtaacatagcacagaacctagtgttctcaacttcccgccctctgcccatttttgctgatgctataaatacttgaattaaatatgggatcttctttgtaaaaaaggcactcagtctactccccaatctcagaaacacatataaaattatattagtccagaatttttatgcttcctctgtcttcttcgtagtgcctaggagggggctgagtacatcatatctgtgaagaaggaaatagctgcacatgtgtttgtaaattccaaagggctatcttacacttaaagcatgctgatgcttaatattggttttaagaattttcagtttgagcatctgaaatgttctcatggcagctattcggaggacattggtttccctaatgctggtgccctgtcaggggccatgtttctgttggaagagaagcacctgctctttgggctggtgtgccagtcttcccttagggaaattggtttgaggagtacaggcactgggatgatttctgagtttttaaatgaatgggcttttattgtaagatgaactgcatgcccctccaggttggtaatcttctaacctgggcctgcagcaacttggacagggacgagggaagcagggctgggagacagcatctccctccagtcaattttccagatgaagccaaataccccattatggtatttgatgatctttatgtacaaaatatttatatacaatgtgccctacaaagatggaagaaaggggcttcatcatgttgatgaggatggaatgttaaatacattaggcaaatggatagatttggtgctagaacaactaaatgatttctaggcttctaatatttatttcctaagagtcatcctctacatagctataaaatgtggtggttggtaacataaactgcaaagcctagggagtaatttcatatttaacctgggcctgcagcaattctaaaaaggacaagggaagaggactggggagagagcatctcccttcaatcagttgtccagatgtagccaaatacctagttagatatctgacagtacacacacacatacacacacgacacttatttacattataccctccaaagatgaaagaaacgaagtcatttaatcatgctgatgaggatgaaagagcttccagttatacactataagcagatggggagctgcagtgctgaactaatcatatgatttctagacttctaaggtttttctcctaaatgtcatctacatgtgccataatagatgttggtgatacaagcccacaagtccaggtgagtgattttacacttaaagtggacctgcacaactctaaaagggggagggagataggcctggggagaagttatctcccttcagtcagttatccagatattgccaaatatctcaacacagtatctggcagaacaaatacatagaaaaatattttatatacattatgccccatcacaatggatagcaaaggattaactgtgcccatgatcatgaaagagctaccacttccacactttgggcagagagggagatgaagtcctaggctaattaaatgatggataggctcctcaagtgtatgtttttctaagggttatcatcaatatgtgcacactcatggaaatgccacctttcaagccactttaaaaacacaggtaataagaaaacaaactgattagtaaaaaacatttgatttcatagactctgttgcatgcaacccaactatttcataaggtaaaaacagtgctatatttttgataatgtcccattatcttgctttaatactatcaacaactgcttgtacaaaagaaacagccatgattgaattctgattctttttttcttgctttctgccagagtttgccaagaactgctttagcccccagcccacagcactgtggggctgcaaggaatgctctatagggtccaggattttaagagtcaaggcaagaatgagagtaagaaaaaaaaaaaaaaaaaggaaaaaggcttacttggagaggcaggtcagggactcagcacttaaacaggtttgtaacaaatccaaagaggagaaaagacatctaagagaaatgttcttcccttcggcaacatgataagcgaaacatatgtataaaaaaatgtataatttcacccagtggtgtgctgatgaatgtttatcaaccagcaatctggagagggagaaaaccccaatttcttacatattgctaatttctgtggtgtaaatatttctaccatggccaatttcaagccactgtagtaacaagaaggtagtgaacatggagttgagaggatacgttcagtagcatactgtttggtaatatttctacatacatacctactagatgtaaataatctaagaggttagaaaatagtaaaatgtaagatttttgagtacagtatttgttacttctgtccttaatataattcattcagttgtaagtgcacatcatttaattttaaataatggctgtattgaacaaccagtttgcaaaattcttgaaaatataacagttggcaagcctgtacaagttgactccaacacatcacacctaaatgggtgaaagggaaggaaaaatcagactgaaaaccataaacattatttactatgttttttaaatagataaggagatgaagccataaactaattaaaggattttcaggggccaaaggtgttagaatattctgcttatggtgttctcaaacattaaaaaaatttcaagataatgagatgtttcaaaggacttcagagacacagatgtgggtacttacaatacaggtaaatgttcaattttacaagggctatcttaaacagattccatgtgttttacaagctaaatagaataatatattaattattttcctattcacttgttttattgctactaggcaactcaggaacactcagctactaaacaaattctggaatttgtttagtaacaaattacagagaaaagaggaaaaaaaagacaatgaattggaagaaagggaggggagaaaggaggaatagagggtgagttgccttgggcagtgtcagaatgtcaccaatcacaacctcaggcactgacagttatcagagttgtgagcttgagccaaaggctgcagtcacctgcttcattagtttagcactgcatttttacaccactacattgaaagattaatgcatactacaatgcaaccatctcacttgtactttcacaggctttgtccttgagatgacatgcatctggataaataattcacatttttctcctgacgtttgcaaatgtctggatggatcatatactgtggacaaaaatctagataattaacctgaatgtttatatttaatccagtgatcttgttacactaaagacaaagcaataaatgcttctaaaatttgccaaaaaatgcaatcatctgcatcagacagccttgattaagatacaatattgttgttttattcaggaatgtactgttttaaaagcttctctcttactaaaatttagaaaatttctatcatgtttgaaaaactttaaaacagctttgtaaatagcctttaaagtcatgttaaagattcaatttatgttgaatagtcagtaaaagtaggtgtgtaattcattttgctacctgtgagtctggcttgatgctacatttgtgggttaataaatagacttctttgctactgttttaaagtgtcataatgttgtcttgctttatgaagatgacactactgatctccaatcaacagggcatgtgcatttactgatttttctggaactaagagagaatttgtgctaaattggtcacattttcacatgcagtgaaagattggcaatactaacttcttatgtggtcagtagaacacttctgatgtatttagcctaactcaaagctatgcatgtaaacagagataggcctctatcataatcacagttacaaacacatattatacactaaattcctttcagtgattaaaaaaacaagttcatgtaagaaagcaagacaacccaataagaaagtggttaaattcattttccatgtcgtcactctctaaaatctgcatcggtccatttgtcaagttgccagaagtgcccatgagcaaataaaacaattgcatatattacaaaatccaagataaataagtagtgctaaaaaagaataacaattaaattattagttatgtggttaacggaaatgaacgaactttgataaaatggtcctgatggggaagaagaagagtttttgtttttcaatggccataccacagtgaaacttcacttctcctcaaggaagtttaccttcggtctgcttcaactctcttcttacgaaccaggtcattattctttgtgatggcagctgccacccttgttcgtggcccttgcttggtaaactggtatccaaacttgaggatccttgaattctcctccagcatctgggcaatttccatctctacagctgttcccaactgctgcctctggttgtcaatcttgatttctgtcaaggtgtcattttctttcagtgcctctaccagggccaggatcccagttccagtgataaaattggattctatgtttagacttgtcaaggtcttgtttactttcagcatgtctgcaaaagcaatggccacagggtcattgctgcgagttgcggccaggctgaacttcttcacgtgagtgttggtctccagagcctttgcaaattccctcagggttggaattggaatgttcttaatgttgttgaggttgacttcttgcaagctaggatcattggctttcatctgctgcaggcttatttccacatttgtgggatttggtggttcctcaaatactggctttactttttcacctttgacaacatttctgacaggtcctttgccacctttattgttggctgtttcttcatcgaactttggattgttgagcaaattgtgtactccaaggacagctgcaagatcatagagttcggtgtcagaggcactggccaaagcttcttccagttctgggtcaagggtcactttttcttctttacgagtttctataggcttttctttagggataaagactctccctttcttttctccagtgaagggcacaaagtcctctctgtctttctgttccaaagcctccttctccaggtacatgaggaggtgctcgcggtcaaaggggccggtggctgccttctgtgtctggtctttctgtcgaaatccagctggcagcatggcactctcaggatctaggtcatctagaacattttccaactgtttcagttcctcttctgagagtttgccaagaagctcatcttcatcaatgttcttgtatttctccagctctttttgaaaggggagtgccatggcttcttataagcctttctcatgggccatgcacatttaaatggtccagtttcctgagacttcagaataccgtccgtgcgctcatcccggagccggctgtgctggccgtcagtccgtcagccccggtggagcggggccgggagaacaggggcggcgccgtggccggggcgagcgcggcgatcaac

SEQ ID NO: 15472 - RNA, 7693 nt, Homo sapiens
  source 1..7693: mol_type = other RNA
gctgggattacaggcatgagccactgggcccagcctaaatagtatatatttttaaatatcctttcagaaaaggccgcttatccagaaccattctgaagacagtaaagaactgctgaagaggaagaaaaaactggctgtgcaatagtcagacctcctctgaacaaagcctcctggagagaaacagctgcagtggaggcattactcacccatgttcagaggcaacggaaacgatttagaatcacaagcttgtcaagtattggagctggaagggaccttagggagcattgaatctactcacttcattttacagatgaaatgaagacaagatagatggagagtcttgcccaaagtcacatagagctggcatccaaatcactattgtttctcaaaaatatcacatggtggcaaatggagcataactctgtggggctggacgacagctaaattcaagcaacatttgttcattaagcacctactatgtacaaggcaccttacaagatggtactgaagatacaaagatggatgagacacagtcctgcctccaagggcttatgaaagtcattggaggccatgcttcaaaacctttcttagcagaaatattactgaccagggctaaggttgctggtgataacaaggcagctgctgccctggagaggtgatctcacaacaggtggcactttctccccttcactatctatcagaactaatgcctgttactcagctgctaggcattaaaattcttgaaaccctaaggacactcttctctcctaggcctccagtcaaacctgaagtcttagcctctcccacccacagcaatgacaggagggcagtagcgctccagaccctcccctcaattcttagtcaactgttcgctttctcccttgtgcccagcctaggccctctgcaaggactgacaatttcccaaggtactgtcaaagtgacccaggaaaatgtcctaccatatacatcgctggtatctaacttccactgccccatcaaccacctctcccacctctacatgggagctgaaataactccagtccctgatgacacacccaagcctcaattacccatactccaaaagatgagaaagatgtaatggttggttagaataaagccgattcaagaggcagtggaaaacagtgatttgataataaaactgatctctcacatttgtacggcgctttccagtttatatagtgtttttatccagttatctgattatattcttaccacaactctgtgaggtagttagtgaagtattattcccattttatagctgaagaaccttaggcttgagagaccaagcggtttgcccaaagttacccagctaaggaagtgtggagccaagtgtccaggtttcttgactccaaatccagtgctcttccccctatatagtctataattggcaggcaattgaatgaattgcccatgatcatatacctgctaagtgttggtgatgggattaggtttcagtctccaaatctgttagtacggtgccccttcaccataccaactaactgggccaatgtgctcagaatgtctaccatggaagagatcagaagaacatctagttagttaactactcttttctatgtctaggtcatcagttctctccttcatcctcccccaagtcaacaatgtatcccaactggcaaagcctctaaaacatgcactattcctagaacagaacccagagtcaggttacaaatttaaacttgcaactcctcttccattggtctactgattattcagtcattgctattacagacagatgggaaagagataagctgagcaaatctcagttctgccattaaacaaatgtaaacctttaatttccatcatccttccccacctcggtcagcaatttgacttcttaactcctgaactacaaagtaaaatccaatctgatctagggttagggagcaataaagcagtgaataatatccctgaagttcttggcgcttttctctggctagtatattacaacaggaggccctatcgtctgattttcatccagtgggctcagctggatgcttccaagcactctcacacctttcctttgtgtgcatctcagtactttagctttaggattggttgagtagcagggatatttgagatgaaagcaataagaggaggtaaagggaagctgcaagtggaaggcagagctaggacctttcctcttagttctctgctcgttaaaatgaaaacagctattattgcatcattagtggaagaggggaaggaagcttcaggatcatgacttaaaacctgactccagaaacacttctactgaatacaggtaacatagcacagaacctagtgttctcaacttcccgccctctgcccatttttgctgatgctataaatacttgaattaaatatgggatcttctttgtaaaaaaggcactcagtctactccccaatctcagaaacacatataaaattatattagtccagaatttttatgcttcctctgtcttcttcgtagtgcctaggagggggctgagtacatcatatctgtgaagaaggaaatagctgcacatgtgtttgtaaattccaaagggctatcttacacttaaagcatgctgatgcttaatattggttttaagaattttcagtttgagcatctgaaatgttctcatggcagctattcggaggacattggtttccctaatgctggtgccctgtcaggggccatgtttctgttggaagagaagcacctgctctttgggctggtgtgccagtcttcccttagggaaattggtttgaggagtacaggcactgggatgatttctgagtttttaaatgaatgggcttttattgtaagatgaactgcatgcccctccaggttggtaatcttctaacctgggcctgcagcaacttggacagggacgagggaagcagggctgggagacagcatctccctccagtcaattttccagatgaagccaaataccccattatggtatttgatgatctttatgtacaaaatatttatatacaatgtgccctacaaagatggaagaaaggggcttcatcatgttgatgaggatggaatgttaaatacattaggcaaatggatagatttggtgctagaacaactaaatgatttctaggcttctaatatttatttcctaagagtcatcctctacatagctataaaatgtggtggttggtaacataaactgcaaagcctagggagtaatttcatatttaacctgggcctgcagcaattctaaaaaggacaagggaagaggactggggagagagcatctcccttcaatcagttgtccagatgtagccaaatacctagttagatatctgacagtacacacacacatacacacacgacacttatttacattataccctccaaagatgaaagaaacgaagtcatttaatcatgctgatgaggatgaaagagcttccagttatacactataagcagatggggagctgcagtgctgaactaatcatatgatttctagacttctaaggtttttctcctaaatgtcatctacatgtgccataatagatgttggtgatacaagcccacaagtccaggtgagtgattttacacttaaagtggacctgcacaactctaaaagggggagggagataggcctggggagaagttatctcccttcagtcagttatccagatattgccaaatatctcaacacagtatctggcagaacaaatacatagaaaaatattttatatacattatgccccatcacaatggatagcaaaggattaactgtgcccatgatcatgaaagagctaccacttccacactttgggcagagagggagatgaagtcctaggctaattaaatgatggataggctcctcaagtgtatgtttttctaagggttatcatcaatatgtgcacactcatggaaatgccacctttcaagccactttaaaaacacaggtaataagaaaacaaactgattagtaaaaaacatttgatttcatagactctgttgcatgcaacccaactatttcataaggtaaaaacagtgctatatttttgataatgtcccattatcttgctttaatactatcaacaactgcttgtacaaaagaaacagccatgattgaattctgattctttttttcttgctttctgccagagtttgccaagaactgctttagcccccagcccacagcactgtggggctgcaaggaatgctctatagggtccaggattttaagagtcaaggcaagaatgagagtaagaaaaaaaaaaaaaaaaaggaaaaaggcttacttggagaggcaggtcagggactcagcacttaaacaggtttgtaacaaatccaaagaggagaaaagacatctaagagaaatgttcttcccttcggcaacatgataagcgaaacatatgtataaaaaaatgtataatttcacccagtggtgtgctgatgaatgtttatcaaccagcaatctggagagggagaaaaccccaatttcttacatattgctaatttctgtggtgtaaatatttctaccatggccaatttcaagccactgtagtaacaagaaggtagtgaacatggagttgagaggatacgttcagtagcatactgtttggtaatatttctacatacatacctactagatgtaaataatctaagaggttagaaaatagtaaaatgtaagatttttgagtacagtatttgttacttctgtccttaatataattcattcagttgtaagtgcacatcatttaattttaaataatggctgtattgaacaaccagtttgcaaaattcttgaaaatataacagttggcaagcctgtacaagttgactccaacacatcacacctaaatgggtgaaagggaaggaaaaatcagactgaaaaccataaacattatttactatgttttttaaatagataaggagatgaagccataaactaattaaaggattttcaggggccaaaggtgttagaatattctgcttatggtgttctcaaacattaaaaaaatttcaagataatgagatgtttcaaaggacttcagagacacagatgtgggtacttacaatacaggtaaatgttcaattttacaagggctatcttaaacagattccatgtgttttacaagctaaatagaataatatattaattattttcctattcacttgttttattgctactaggcaactcaggaacactcagctactaaacaaattctggaatttgtttagtaacaaattacagagaaaagaggaaaaaaaagacaatgaattggaagaaagggaggggagaaaggaggaatagagggtgagttgccttgggcagtgtcagaatgtcaccaatcacaacctcaggcactgacagttatcagagttgtgagcttgagccaaaggctgcagtcacctgcttcattagtttagcactgcatttttacaccactacattgaaagattaatgcatactacaatgcaaccatctcacttgtactttcacaggctttgtccttgagatgacatgcatctggataaataattcacatttttctcctgacgtttgcaaatgtctggatggatcatatactgtggacaaaaatctagataattaacctgaatgtttatatttaatccagtgatcttgttacactaaagacaaagcaataaatgcttctaaaatttgccaaaaaatgcaatcatctgcatcagacagccttgattaagatacaatattgttgttttattcaggaatgtactgttttaaaagcttctctcttactaaaatttagaaaatttctatcatgtttgaaaaactttaaaacagctttgtaaatagcctttaaagtcatgttaaagattcaatttatgttgaatagtcagtaaaagtaggtgtgtaattcattttgctacctgtgagtctggcttgatgctacatttgtgggttaataaatagacttctttgctactgttttaaagtgtcataatgttgtcttgctttatgaagatgacactactgatctccaatcaacagggcatgtgcatttactgatttttctggaactaagagagaatttgtgctaaattggtcacattttcacatgcagtgaaagattggcaatactaacttcttatgtggtcagtagaacacttctgatgtatttagcctaactcaaagctatgcatgtaaacagagataggcctctatcataatcacagttacaaacacatattatacactaaattcctttcagtgattaaaaaaacaagttcatgtaagaaagcaagacaacccaataagaaagtggttaaattcattttccatgtcgtcactctctaaaatctgcatcggtccatttgtcaagttgccagaagtgcccatgagcaaataaaacaattgcatatattacaaaatccaagataaataagtagtgctaaaaaagaataacaattaaattattagttatgtggttaacggaaatgaacgaactttgataaaatggtcctgatggggaagaagaagagtttttgtttttcaatggccataccacagtgaaacttcacttctcctcaaggaagtttaccttcggtctgcttcaactctcttcttacgaaccaggtcattattctttgtgatggcagctgccacccttgttcgtggcccttgcttggtaaactggtatccaaacttgaggatccttgaattctcctccagcatctgggcaatttccatctctacagctgttcccaactgctgcctctggttgtcaatcttgatttctgtcaaggtgtcattttctttcagtgcctctaccagggccaggatcccagttccagtgataaaattggattctatgtttagacttgtcaaggtcttgtttactttcagcatgtctgcaaaagccttaatgttgttgaggttgacttcttgcaagctaggatcattggctttcatctgctgcaggcttatttccacatttgtgggatttggtggttcctcaaatactggctttactttttcacctttgacaacatttctgacaggtcctttgccacctttattgttggctgtttcttcatcgaactttggattgttgagcaaattgtgtactccaaggacagctgcaagatcatagagttcggtgtcagaggcactggccaaagcttcttccagttctgggtcaagggtcactttttcttctttacgagtttctataggcttttctttagggataaagactctccctttcttttctccagtgaagggcacaaagtcctctctgtctttctgttccaaagcctccttctccaggtacatgaggaggtgctcgcggtcaaaggggccggtggctgccttctgtgtctggtctttctgtcgaaatccagctggcagcatggcactctcaggatctaggtcatctagaacattttccaactgtttcagttcctcttctgagagtttgccaagaagctcatcttcatcaatgttcttgtatttctccagctctttttgaaaggggagtgccatggcttcttataagcctttctcatgggccatgcacatttaaatggtccagtttcctgagacttcagaataccgtccgtgcgctcatcccggagccggctgtgctggccgtcagtccgtcagccccggtggagcggggccgggagaacaggggcggcgccgtggccggggcgagcgcggcgatcaac

SEQ ID NO: 15473 - RNA, 7692 nt, Homo sapiens
  source 1..7692: mol_type = other RNA
gctgggattacaggcatgagccactgggcccagcctaaatagtatatatttttaaatatcctttcagaaaaggccgcttatccagaaccattctgaagacagtaaagaactgctgaagaggaagaaaaaactggctgtgcaatagtcagacctcctctgaacaaagcctcctggagagaaacagctgcagtggaggcattactcacccatgttcagaggcaacggaaacgatttagaatcacaagcttgtcaagtattggagctggaagggaccttagggagcattgaatctactcacttcattttacagatgaaatgaagacaagatagatggagagtcttgcccaaagtcacatagagctggcatccaaatcactattgtttctcaaaaatatcacatggtggcaaatggagcataactctgtggggctggacgacagctaaattcaagcaacatttgttcattaagcacctactatgtacaaggcaccttacaagatggtactgaagatacaaagatggatgagacacagtcctgcctccaagggcttatgaaagtcattggaggccatgcttcaaaacctttcttagcagaaatattactgaccagggctaaggttgctggtgataacaaggcagctgctgccctggagaggtgatctcacaacaggtggcactttctccccttcactatctatcagaactaatgcctgttactcagctgctaggcattaaaattcttgaaaccctaaggacactcttctctcctaggcctccagtcaaacctgaagtcttagcctctcccacccacagcaatgacaggagggcagtagcgctccagaccctcccctcaattcttagtcaactgttcgctttctcccttgtgcccagcctaggccctctgcaaggactgacaatttcccaaggtactgtcaaagtgacccaggaaaatgtcctaccatatacatcgctggtatctaacttccactgccccatcaaccacctctcccacctctacatgggagctgaaataactccagtccctgatgacacacccaagcctcaattacccatactccaaaagatgagaaagatgtaatggttggttagaataaagccgattcaagaggcagtggaaaacagtgatttgataataaaactgatctctcacatttgtacggcgctttccagtttatatagtgtttttatccagttatctgattatattcttaccacaactctgtgaggtagttagtgaagtattattcccattttatagctgaagaaccttaggcttgagagaccaagcggtttgcccaaagttacccagctaaggaagtgtggagccaagtgtccaggtttcttgactccaaatccagtgctcttccccctatatagtctataattggcaggcaattgaatgaattgcccatgatcatatacctgctaagtgttggtgatgggattaggtttcagtctccaaatctgttagtacggtgccccttcaccataccaactaactgggccaatgtgctcagaatgtctaccatggaagagatcagaagaacatctagttagttaactactcttttctatgtctaggtcatcagttctctccttcatcctcccccaagtcaacaatgtatcccaactggcaaagcctctaaaacatgcactattcctagaacagaacccagagtcaggttacaaatttaaacttgcaactcctcttccattggtctactgattattcagtcattgctattacagacagatgggaaagagataagctgagcaaatctcagttctgccattaaacaaatgtaaacctttaatttccatcatccttccccacctcggtcagcaatttgacttcttaactcctgaactacaaagtaaaatccaatctgatctagggttagggagcaataaagcagtgaataatatccctgaagttcttggcgcttttctctggctagtatattacaacaggaggccctatcgtctgattttcatccagtgggctcagctggatgcttccaagcactctcacacctttcctttgtgtgcatctcagtactttagctttaggattggttgagtagcagggatatttgagatgaaagcaataagaggaggtaaagggaagctgcaagtggaaggcagagctaggacctttcctcttagttctctgctcgttaaaatgaaaacagctattattgcatcattagtggaagaggggaaggaagcttcaggatcatgacttaaaacctgactccagaaacacttctactgaatacaggtaacatagcacagaacctagtgttctcaacttcccgccctctgcccatttttgctgatgctataaatacttgaattaaatatgggatcttctttgtaaaaaaggcactcagtctactccccaatctcagaaacacatataaaattatattagtccagaatttttatgcttcctctgtcttcttcgtagtgcctaggagggggctgagtacatcatatctgtgaagaaggaaatagctgcacatgtgtttgtaaattccaaagggctatcttacacttaaagcatgctgatgcttaatattggttttaagaattttcagtttgagcatctgaaatgttctcatggcagctattcggaggacattggtttccctaatgctggtgccctgtcaggggccatgtttctgttggaagagaagcacctgctctttgggctggtgtgccagtcttcccttagggaaattggtttgaggagtacaggcactgggatgatttctgagtttttaaatgaatgggcttttattgtaagatgaactgcatgcccctccaggttggtaatcttctaacctgggcctgcagcaacttggacagggacgagggaagcagggctgggagacagcatctccctccagtcaattttccagatgaagccaaataccccattatggtatttgatgatctttatgtacaaaatatttatatacaatgtgccctacaaagatggaagaaaggggcttcatcatgttgatgaggatggaatgttaaatacattaggcaaatggatagatttggtgctagaacaactaaatgatttctaggcttctaatatttatttcctaagagtcatcctctacatagctataaaatgtggtggttggtaacataaactgcaaagcctagggagtaatttcatatttaacctgggcctgcagcaattctaaaaaggacaagggaagaggactggggagagagcatctcccttcaatcagttgtccagatgtagccaaatacctagttagatatctgacagtacacacacacatacacacacgacacttatttacattataccctccaaagatgaaagaaacgaagtcatttaatcatgctgatgaggatgaaagagcttccagttatacactataagcagatggggagctgcagtgctgaactaatcatatgatttctagacttctaaggtttttctcctaaatgtcatctacatgtgccataatagatgttggtgatacaagcccacaagtccaggtgagtgattttacacttaaagtggacctgcacaactctaaaagggggagggagataggcctggggagaagttatctcccttcagtcagttatccagatattgccaaatatctcaacacagtatctggcagaacaaatacatagaaaaatattttatatacattatgccccatcacaatggatagcaaaggattaactgtgcccatgatcatgaaagagctaccacttccacactttgggcagagagggagatgaagtcctaggctaattaaatgatggataggctcctcaagtgtatgtttttctaagggttatcatcaatatgtgcacactcatggaaatgccacctttcaagccactttaaaaacacaggtaataagaaaacaaactgattagtaaaaaacatttgatttcatagactctgttgcatgcaacccaactatttcataaggtaaaaacagtgctatatttttgataatgtcccattatcttgctttaatactatcaacaactgcttgtacaaaagaaacagccatgattgaattctgattctttttttcttgctttctgccagagtttgccaagaactgctttagcccccagcccacagcactgtggggctgcaaggaatgctctatagggtccaggattttaagagtcaaggcaagaatgagagtaagaaaaaaaaaaaaaaaaaggaaaaaggcttacttggagaggcaggtcagggactcagcacttaaacaggtttgtaacaaatccaaagaggagaaaagacatctaagagaaatgttcttcccttcggcaacatgataagcgaaacatatgtataaaaaaatgtataatttcacccagtggtgtgctgatgaatgtttatcaaccagcaatctggagagggagaaaaccccaatttcttacatattgctaatttctgtggtgtaaatatttctaccatggccaatttcaagccactgtagtaacaagaaggtagtgaacatggagttgagaggatacgttcagtagcatactgtttggtaatatttctacatacatacctactagatgtaaataatctaagaggttagaaaatagtaaaatgtaagatttttgagtacagtatttgttacttctgtccttaatataattcattcagttgtaagtgcacatcatttaattttaaataatggctgtattgaacaaccagtttgcaaaattcttgaaaatataacagttggcaagcctgtacaagttgactccaacacatcacacctaaatgggtgaaagggaaggaaaaatcagactgaaaaccataaacattatttactatgttttttaaatagataaggagatgaagccataaactaattaaaggattttcaggggccaaaggtgttagaatattctgcttatggtgttctcaaacattaaaaaaatttcaagataatgagatgtttcaaaggacttcagagacacagatgtgggtacttacaatacaggtaaatgttcaattttacaagggctatcttaaacagattccatgtgttttacaagctaaatagaataatatattaattattttcctattcacttgttttattgctactaggcaactcaggaacactcagctactaaacaaattctggaatttgtttagtaacaaattacagagaaaagaggaaaaaaaagacaatgaattggaagaaagggaggggagaaaggaggaatagagggtgagttgccttgggcagtgtcagaatgtcaccaatcacaacctcaggcactgacagttatcagagttgtgagcttgagccaaaggctgcagtcacctgcttcattagtttagcactgcatttttacaccactacattgaaagattaatgcatactacaatgcaaccatctcacttgtactttcacaggctttgtccttgagatgacatgcatctggataaataattcacatttttctcctgacgtttgcaaatgtctggatggatcatatactgtggacaaaaatctagataattaacctgaatgtttatatttaatccagtgatcttgttacactaaagacaaagcaataaatgcttctaaaatttgccaaaaaatgcaatcatctgcatcagacagccttgattaagatacaatattgttgttttattcaggaatgtactgttttaaaagcttctctcttactaaaatttagaaaatttctatcatgtttgaaaaactttaaaacagctttgtaaatagcctttaaagtcatgttaaagattcaatttatgttgaatagtcagtaaaagtaggtgtgtaattcattttgctacctgtgagtctggcttgatgctacatttgtgggttaataaatagacttctttgctactgttttaaagtgtcataatgttgtcttgctttatgaagatgacactactgatctccaatcaacagggcatgtgcatttactgatttttctggaactaagagagaatttgtgctaaattggtcacattttcacatgcagtgaaagattggcaatactaacttcttatgtggtcagtagaacacttctgatgtatttagcctaactcaaagctatgcatgtaaacagagataggcctctatcataatcacagttacaaacacatattatacactaaattcctttcagtgattaaaaaaacaagttcatgtaagaaagcaagacaacccaataagaaagtggttaaattcattttccatgtcgtcactctctaaaatctgcatcggtccatttgtcaagttgccagaagtgcccatgagcaaataaaacaattgcatatattacaaaatccaagataaataagtagtgctaaaaaagaataacaattaaattattagttatgtggttaacggaaatgaacgaactttgataaaatggtcctgatggggaagaagaagagtttttgtttttcaatggccataccacagtgaaacttcacttctcctcaaggaagtttaccttcggtctgcttcaactctcttcttacgaactggttgtcaatcttgatttctgtcaaggtgtcattttctttcagtgcctctaccagggccaggatcccagttccagtgataaaattggattctatgtttagacttgtcaaggtcttgtttactttcagcatgtctgcaaaagcaatggccacagggtcattgctgcgagttgcggccaggctgaacttcttcacgtgagtgttggtctccagagcctttgcaaattccctcagggttggaattggaatgttcttaatgttgttgaggttgacttcttgcaagctaggatcattggctttcatctgctgcaggcttatttccacatttgtgggatttggtggttcctcaaatactggctttactttttcacctttgacaacatttctgacaggtcctttgccacctttattgttggctgtttcttcatcgaactttggattgttgagcaaattgtgtactccaaggacagctgcaagatcatagagttcggtgtcagaggcactggccaaagcttcttccagttctgggtcaagggtcactttttcttctttacgagtttctataggcttttctttagggataaagactctccctttcttttctccagtgaagggcacaaagtcctctctgtctttctgttccaaagcctccttctccaggtacatgaggaggtgctcgcggtcaaaggggccggtggctgccttctgtgtctggtctttctgtcgaaatccagctggcagcatggcactctcaggatctaggtcatctagaacattttccaactgtttcagttcctcttctgagagtttgccaagaagctcatcttcatcaatgttcttgtatttctccagctctttttgaaaggggagtgccatggcttcttataagcctttctcatgggccatgcacatttaaatggtccagtttcctgagacttcagaataccgtccgtgcgctcatcccggagccggctgtgctggccgtcagtccgtcagccccggtggagcggggccgggagaacaggggcggcgccgtggccggggcgagcgcggcgatcaacaggcggctcccggccgggcgcggcgccggggcgcgc

SEQ ID NO: 15474 - RNA, 6743 nt, Homo sapiens
  source 1..6743: mol_type = other RNA
gctgggattacaggcatgagccactgtaccaggctgagtccacacttctaagcttgctgttgctctcagacttgcagaacaacctattaaacagaagtaggtaaaagttgagaaagggaagtggccaccacagaaccagttctgctgagaacgaggactcgagtcaggctatgctaccctccttccatggccatgggaaaaaggggtgtgtgctgttggtgtgagagatctggatcttaacagatcagacttaaactaatttgcccatgatgaccgtgtggatttggagggacctgggaatctcacagacctatgggatgtcccagtgatatgtcctgggcttcataccagccctgccctgcctgacaagttggatgaaaactgataaaggacttgtcatagcttcagatggcaaaaccaggccaggccagaatgaaaaaggagaaggaatttaacatgggcaaatgccaagctctgcatttaactaaccaaggctgcttggcgtgaacaaaactgagacagagcaatgcatggagaaaagggttgggcatttgtgggctacaagcttggcatgacatggatgcaaatgtcaatgggtgcacccccagatgcctgtgactccctctggtggtttctgtgcacaacttcccccaaaataggccctacgactccagcagaaacctaccctggggctcctagagcttcctagcctgcctgccagagagcagaagtgcctggaggctacatcttcacccctgggtagtccttactctgaggtgggactgcatccagggctcccctttagggtctgacttggactgaaatcacaccctgccttgccttctgcccctcccttaacttgctctcccctccctaataactccagcatcctcatctcagcagaagcttctggggaacccagcccaagatgagtggtgagggctagggtagccctcctcaatgcactctgggaactacattttcagaagccccagccagagggccaagtcccaggcagggtgcaaagctgtggggcgaggaacctggaaagaggctctgaacaagggacttttaaggaagtgggatgtgggctgtgatcacagccaagctggcagggtaagaggtggcccctgaatgtggctatgagaggggtgcccaacactaccagcctgtgtgctgagcactaactcagtgccaggcactacttgggttattctatttaatctccacaccaagcatgtgaaggaggcaccattgtcatccccatcttacagatgaggaagatgatcaaggcttgtaacttgcccaagatcacatggctataggtgtggatcctatatatccagattcaaactccagctttagcccactaagctacggtggccaaccccagcccaaagtgttgggacctgcgtgtagaagaccccttcagcccttgtaaagttaggatctagcatgtctaaggggacagagacccaatccaggtgacacaggaggtaagatcacagtggaacaggccatccctgcttttccaccaccaccagcactgtgacctcagaccagctctactctatgagtttcttgtgacagtgatggcagcctggggccagacaagggatgcgtgtcttgtgtcctggacacaagacaggcaggcccagaggggacaagctatatgaagagaggcttcagctgtcgggggtcctgaatgccatggaaggagagcaggtgggcagaagcagggagcccctggagcagacagaggggggattcctgctgaggcaaggggctctaggactccagggtttatgctccaaagaacagaatttaccaggacaaaataaacaagaccagtcaggaccgatgccccatccctgctggggtctggcaaagctctcacctccaaatttgtatctgttttgaattcaaagccaaacaaacacatcaacagtgaactccaacacctcccagagcagggcctgaaagggacccagaaagtctggccagaaatctagagtccaaggggaggagatctgtaaactaaaccgctggccatgctctggggccctaaaccactgcaggcatcagggctgttccaggagagggcacagcaaagggggttgggaggggtctccagttccaatcagaaatgaggctgcagtcacttcaggtagacctgtcagcagcagctgtgcaactgggctagggagacaaggatcgtggtttagccaggagaatcatctggggccccagccaagacacaggtgttggatttcagcaccgctctgcaaatactcatctcagtgacgatgaggtgagtgggagcttggctgagcccagcccggcctgccatcctggcaagccagggcagcatggaggtagcacagagtggcacccagccagcgtgaatgcataagaatctgcacgtgacacagaagaaagtctcttcatgaagtaggtttcactggtcccagccaaaccctgtggcaggtggccctttctgcacctgctgaacatgccattcaccttgacccaggtagtggcctcaccctcctcttgctcaaactggaaacctcagcatcctgaaatgcctcctccccaaatccattgcacacatgtgtgcctgtgtatgcgtgtgtgtgcacgtgtatgaacccagcccccagctgcccactccattgcccctaaacaggcccctccttggtgtcacctggcacatctccactggaagccaaatggatatttctaaactgaaatctggtcccacctcagaaccccttccacagttcccttaaagttcctttcctcatttacatcaggatcttcacaatggggacccctggtcacctcccaacccaacaaacgctccaaatgagccgccactgcagaaactcattatggcccaggcaggacaggcacatccaagtatctgaccaggctgttccatctgccaggcaggtcctgccctctctccacccacctgtctaacccctgcatcctcaagaccctacttagctatggccctgtgtgaaaggtccctccccatgcacccacagccatttgttctctctcatgtggccctaacaggctggggttcctggagactccatggggagccaggcatgaagatggcatatacccatgtgtcactccccagaacgtgagctgcctgccctggcaccatacacaaagggactgacagccccagaatcccaaggggtgcacctatgcatatgggaaaggcatgtttacgggtgagaatggtccatcgttgggcttcaggaggcatctgacctgacgcacgcctttgtcactttgtccttgtggcctgttgaaatgccactcctgctttacaaattcaccaactgttgcatgagtcatttccacctcaatgagtaccaggtccttgaggatggggaaaagtaagccaccactgtgggggtcctgggctcctaggtgcagaagaggctccagaaacaggccaggtcgtgggccatgaccccacactagccctctggtccctcacacgggtggattggggggctgtgtcacgggatcttaggatcttcaagacaaagacccaggacaagaacacaagcccactcccattcttcacaggcctcgagaaatctttgggcaatgaagtcagactgtgccaaagcccatgtttctgtctctccaaggcccctggcccccactgcctagcctaggtcaggtcatgtgggcaagcgagcccccacagcctcacagcccctaccccagggccagggcaaactcctgccctgtccccctccattcctgccctccctccttccacaaactgcaccagctggggagaaatccttcagccgacagaatgaggtgaaaatagtgcaattttaggctttgtaactgagattagggcaggtggccacccattctccccttcctcaggccagcctctgacacaatgaccctggaagcctggcagccctccgtaatggtcagcatcctcccctgccatccccaacccacaccatgagctcagccagggcaggggcagcctctgtctcattcaccacagaatccacagaacccagcacagagtatgagctcagtaaattctcctcatacatgactgcactgactggaccgggcacatgctacagggcaacacccacggctcagctggccctggctttggatctcagtcccacctcttcaagctgtccagcgtggggcacatcggctacagccttgccaaatgaaggcttgccaggatgaagaggtgaagacaggacaagcacagtatgtggcacacaggaggcctctgataacatcagtccccttccctaaagacctgggcagtccctgtcactggggcctcacatttcatgtcgagaattcactatttctcagcactgatttcaaataaagccaccaagagtctgacgaggcaacatggcagagttctgagggtggagtgaacaaaaggtcattttttacagaaaactcaggatctcccctctgcacagtgctaaagccctgtctcaaagttcagagcccggaaggtgcagagatgtggcccttggaaatcaagcccttaagaaaacagcccagctgtgtagggccggaagccccaggctgcagtcctgtggtctggaggcagccaatattcaggtgagagatgtgcccagctgccggtgggtccagggggcacggagcccccaccgtccctggcccaggtctaggactaagtcagtgggcccaggccagctccaagggccacagctcctcactcgggggccgcgccggagcagccgcagcagctggggcgccgcagggactgcatgacagcccgcagtggccccctccggccctccacagacaggctgtcctcgctggcgggcgcccgctgcagctgctcaaactgcatctccaggtgcttctggatggccacaccgagcacctccaggtccaccgcagctccgtacacctcccatgtcatgccctcagcatcccatcgcacatcccgcacaggggacggcacctcctccaggctggaccccagagttacctctgggaacacatgcagggctgcaggcgcttccagggacggactggtggccacagccttgcaggccgccactggggccgcctgcacaccagcatcctgggctgacagcggggatgcctctgcaggggccaagtcattggctgaggtcatggtccacacatctttggtcctagagccaggctctgggactaacccagcgggaccccaaaggtgggcacagcaatgggaatgcccagggagccccccagacaacctacagtggatcttcaccccatgctgagcctgcagcccagactcgctcactgacgccactagtttgggaaaggccaggatccctgtggcaggtagggcatggcagcagccaccagccctcacctccctcatgccacagagtagagcagctgggggcagagcatggcaggtggtggtagccagctgttcagcagctttgggctcagcctgggcactgctgctgtgggcagttgtgtcccccaggtctagtggtggcactgacaactgactcgcccccagcatccaggctgagttagaagtctcatcctcaggagccaggtccctttccaggcctgcaggggcctggccaccctggccagaagtaccacctggctgcagctgagccctgtggacagggctgctgccaagggctgagcagctgagactggccttccgagcaccactgtgtccccgcatctgggtgctacggaccaggtctgaatggctcctctgcatagcagcagcactaggggcccgcaggcgacacaggtcactgccgcccatggtggacacattgcccacagtgctgctccaccagtggcctccagcactgggtcgcgccttggggccagaggcccgtgctggcttcatgctctcaggcgggttcccctcttcctccggggcctggggtctggtgctggcctcgcccagctgggcctgccacacggtgctgctggcagtcttgcggagctctggcctctgttcccggccttcacccagcaggctggaagagctctgggacaggggctgaaggcgggggctcaggggtgcccagggacccggctcggggcggctggagctcatggctgcctctagctccaggggcaaggagaggccccatgcatcagctttttccatgagggactcattcagcatctggtcattgattccacagcatctcctgagcccctactgcgtgcccagctgtagggccacagaggagggcactgagtgccaaaaatggggtctgagggagggcaccaccaaggcaggagagctcacggagggtgagagatgagaaaaggcttcctggaggaccagccacgtaagtcaggccttaatgttctctctcctgccccatttgatgccgaagttgctatggttgtggccgatgtcccgtggccaatgccaggctgtcctgctgcctcaggttccacctgtcagcaactctcaaggaccaggcaggaatgcacacagcacaaacccccattgcacagtggggatacagcaccctccaggaggtggtttaatccaccccagagtgaacggggcctgataggaacactcagggccaactctgggcaaagcagcaggcagcattccacgccccgcattgaggtctccgcgccggcggctacccctttcctctcgccttctccatcctagctccgcctctcac

SEQ ID NO: 15475 - RNA, 7331 nt, Homo sapiens
  source 1..7331: mol_type = other RNA
gctgggattacaggcatgagccactgtaccaggctgagtccacacttctaagcttgctgttgctctcagacttgcagaacaacctattaaacagaagtaggtaaaagttgagaaagggaagtggccaccacagaaccagttctgctgagaacgaggactcgagtcaggctatgctaccctccttccatggccatgggaaaaaggggtgtgtgctgttggtgtgagagatctggatcttaacagatcagacttaaactaatttgcccatgatgaccgtgtggatttggagggacctgggaatctcacagacctatgggatgtcccagtgatatgtcctgggcttcataccagccctgccctgcctgacaagttggatgaaaactgataaaggacttgtcatagcttcagatggcaaaaccaggccaggccagaatgaaaaaggagaaggaatttaacatgggcaaatgccaagctctgcatttaactaaccaaggctgcttggcgtgaacaaaactgagacagagcaatgcatggagaaaagggttgggcatttgtgggctacaagcttggcatgacatggatgcaaatgtcaatgggtgcacccccagatgcctgtgactccctctggtggtttctgtgcacaacttcccccaaaataggccctacgactccagcagaaacctaccctggggctcctagagcttcctagcctgcctgccagagagcagaagtgcctggaggctacatcttcacccctgggtagtccttactctgaggtgggactgcatccagggctcccctttagggtctgacttggactgaaatcacaccctgccttgccttctgcccctcccttaacttgctctcccctccctaataactccagcatcctcatctcagcagaagcttctggggaacccagcccaagatgagtggtgagggctagggtagccctcctcaatgcactctgggaactacattttcagaagccccagccagagggccaagtcccaggcagggtgcaaagctgtggggcgaggaacctggaaagaggctctgaacaagggacttttaaggaagtgggatgtgggctgtgatcacagccaagctggcagggtaagaggtggcccctgaatgtggctatgagaggggtgcccaacactaccagcctgtgtgctgagcactaactcagtgccaggcactacttgggttattctatttaatctccacaccaagcatgtgaaggaggcaccattgtcatccccatcttacagatgaggaagatgatcaaggcttgtaacttgcccaagatcacatggctataggtgtggatcctatatatccagattcaaactccagctttagcccactaagctacggtggccaaccccagcccaaagtgttgggacctgcgtgtagaagaccccttcagcccttgtaaagttaggatctagcatgtctaaggggacagagacccaatccaggtgacacaggaggtaagatcacagtggaacaggccatccctgcttttccaccaccaccagcactgtgacctcagaccagctctactctatgagtttcttgtgacagtgatggcagcctggggccagacaagggatgcgtgtcttgtgtcctggacacaagacaggcaggcccagaggggacaagctatatgaagagaggcttcagctgtcgggggtcctgaatgccatggaaggagagcaggtgggcagaagcagggagcccctggagcagacagaggggggattcctgctgaggcaaggggctctaggactccagggtttatgctccaaagaacagaatttaccaggacaaaataaacaagaccagtcaggaccgatgccccatccctgctggggtctggcaaagctctcacctccaaatttgtatctgttttgaattcaaagccaaacaaacacatcaacagtgaactccaacacctcccagagcagggcctgaaagggacccagaaagtctggccagaaatctagagtccaaggggaggagatctgtaaactaaaccgctggccatgctctggggccctaaaccactgcaggcatcagggctgttccaggagagggcacagcaaagggggttgggaggggtctccagttccaatcagaaatgaggctgcagtcacttcaggtagacctgtcagcagcagctgtgcaactgggctagggagacaaggatcgtggtttagccaggagaatcatctggggccccagccaagacacaggtgttggatttcagcaccgctctgcaaatactcatctcagtgacgatgaggtgagtgggagcttggctgagcccagcccggcctgccatcctggcaagccagggcagcatggaggtagcacagagtggcacccagccagcgtgaatgcataagaatctgcacgtgacacagaagaaagtctcttcatgaagtaggtttcactggtcccagccaaaccctgtggcaggtggccctttctgcacctgctgaacatgccattcaccttgacccaggtagtggcctcaccctcctcttgctcaaactggaaacctcagcatcctgaaatgcctcctccccaaatccattgcacacatgtgtgcctgtgtatgcgtgtgtgtgcacgtgtatgaacccagcccccagctgcccactccattgcccctaaacaggcccctccttggtgtcacctggcacatctccactggaagccaaatggatatttctaaactgaaatctggtcccacctcagaaccccttccacagttcccttaaagttcctttcctcatttacatcaggatcttcacaatggggacccctggtcacctcccaacccaacaaacgctccaaatgagccgccactgcagaaactcattatggcccaggcaggacaggcacatccaagtatctgaccaggctgttccatctgccaggcaggtcctgccctctctccacccacctgtctaacccctgcatcctcaagaccctacttagctatggccctgtgtgaaaggtccctccccatgcacccacagccatttgttctctctcatgtggccctaacaggctggggttcctggagactccatggggagccaggcatgaagatggcatatacccatgtgtcactccccagaacgtgagctgcctgccctggcaccatacacaaagggactgacagccccagaatcccaaggggtgcacctatgcatatgggaaaggcatgtttacgggtgagaatggtccatcgttgggcttcaggaggcatctgacctgacgcacgcctttgtcactttgtccttgtggcctgttgaaatgccactcctgctttacaaattcaccaactgttgcatgagtcatttccacctcaatgagtaccaggtccttgaggatggggaaaagtaagccaccactgtgggggtcctgggctcctaggtgcagaagaggctccagaaacaggccaggtcgtgggccatgaccccacactagccctctggtccctcacacgggtggattggggggctgtgtcacgggatcttaggatcttcaagacaaagacccaggacaagaacacaagcccactcccattcttcacaggcctcgagaaatctttgggcaatgaagtcagactgtgccaaagcccatgtttctgtctctccaaggcccctggcccccactgcctagcctaggtcaggtcatgtgggcaagcgagcccccacagcctcacagcccctaccccagggccagggcaaactcctgccctgtccccctccattcctgccctccctccttccacaaactgcaccagctggggagaaatccttcagccgacagaatgaggtgaaaatagtgcaattttaggctttgtaactgagattagggcaggtggccacccattctccccttcctcaggccagcctctgacacaatgaccctggaagcctggcagccctccgtaatggtcagcatcctcccctgccatccccaacccacaccatgagctcagccagggcaggggcagcctctgtctcattcaccacagaatccacagaacccagcacagagtatgagctcagtaaattctcctcatacatgactgcactgactggaccgggcacatgctacagggcaacacccacggctcagctggccctggctttggatctcagtcccacctcttcaagctgtccagcgtggggcacatcggctacagccttgccaaatgaaggcttgccaggatgaagaggtgaagacaggacaagcacagtatgtggcacacaggaggcctctgataacatcagtccccttccctaaagacctgggcagtccctgtcactggggcctcacatttcatgtcgagaattcactatttctcagcactgatttcaaataaagccaccaagagtctgacgaggcaacatggcagagttctgagggtggagtgaacaaaaggtcattttttacagaaaactcaggatctcccctctgcacagtgctaaagccctgtctcaaagttcagagcccggaaggtgcagagatgtggcccttggaaatcaagcccttaagaaaacagcccagctgtgtagggccggaagccccaggctgcagtcctgtggtctggaggcagccaatattcaggtgagagatgtgcccagctgccggtgggtccagggggcacggagcccccaccgtccctggcccaggtctaggactaagtcagtgggcccaggccagctccaagggccacagctcctcactcgggggccgcgccggagcagccgcagcagctggggcgccgcagggactgcatgacagcccgcagtggccccctccggccctccacagacaggctgtcctcgctggcgggcgcccgctgcagctgctcaaactgcatctccaggtgcttctggatggccacaccgagcacctccaggtccaccgcagctccgtacacctcccatgtcatgccctcagcatcccatcgcacatcccgcacaggggacggcacctcctccaggctggaccccagagttacctctgggaacacatgcagggctgcaggcgcttccagggacggactggtggccacagccttgcaggccgccactggggccgcctgcacaccagcatcctgggctgacagcggggatgcctctgcaggggccaagtcattggctgaggtcatggtccacacatctttggtcctagagccaggctctgggactaacccagcgggaccccaaaggtgggcacagcaatgggaatgcccagggagccccccagacaacctacagtggatcttcaccccatgctgagcctgcagcccagactcgctcactgacgccactagtttgggaaaggccaggatccctgtggcaggtagggcatggcagcagccaccagccctcacctccctcatgccacagagtagagcagctgggggcagagcatggcaggtggtggtagccagctgttcagcagctttgggctcagcctgggcactgctgctgtgggcagttgtgtcccccaggtctagtggtggcactgacaactgactcgcccccagcatccaggctgagttagaagtctcatcctcaggagccaggtccctttccaggcctgcaggggcctggccaccctggccagaagtaccacctggctgcagctgagccctgtggacagggctgctgccaagggctgagcagctgagactggccttccgagcaccactgtgtccccgcatctgggtgctacggaccaggtctgaatggctcctctgcatagcagcagcactaggggcccgcaggcgacacaggtcactgccgcccatggtggacacattgcccacagtgctgctccaccagtggcctccagcactgggtcgcgccttggggccagaggcccgtgctggcttcatgctctcaggcgggttcccctcttcctccggggcctggggtctggtgctggcctcgcccagctgggcctgccacacggtgctgctggcagtcttgcggagctctggcctctgttcccggccttcacccagcaggctggaagagctctgggacaggggctgaaggcgggggctcaggggtgcccagggacccggctcggggcggctggagctcatggctgcctctagctccaggggcaaggagaggccccatgcatcagctttttccatgagggactcattcagcatctggtcattgattccacagcatctcctgagcccctactgcgtgcccagctgtagggctagggaacatgggattcattcagacctttctgtacccctgatgtgtcgtcggcactcagaggattatctgctgtgtgcctgaccaagagaacaagcaaatacaagaacacacccacagaggagggcactgagtgccaaaaatggggtctgagggagggcaccaccaaggcaggagagctcacggagggtgagagatgagaaaaggcttcctggaggaccagccacgtaagtcaggcaggtggacccctaacttctttgagcctcagtttcttcaatcttaatgttctctctcctgccccatttgatgccgaagttgctatggttgtggccgatgtcccgtggccaatgccaggctgtcctgctgcctcaggttccacctgtcagcaactctcaaggaccaggcaggaatgcacacagcacaaacccccattgcacagtggggatacagcaccctccaggaggtggtttaatccaccccagagtgaacggggcctgataggaacactcagggccaactctgggcaaagcagcaggcagcattcctaaagggagggtttggaggagacaaaacctgcccttcacaatgaacgtgccttaagggctacatgccccgggtcacaagctgtgccaggaaagggttctggggtaactgtggggtcagtggccccatggatgaggctctgctcaccaggaagaggcctaggcgcccaacagcccctgagcttcctcccctggggaggatttgcccacaatccctggggggcacctaggtggagagggtgccccggcctagaagcagcctaggcggccggtgtgtccctatctgcacgctcacaagcactcatgccccagcctgggacacacaggcccgtatgcagtaacagcgtctacccagctgcactctgcacgccaagcacaggccgcccctgctgcggggccaaaggcctgaaagcaccgcaccacgcagcctcgcccagaatagctcccctcccgcccctcctgcacaaagcccacccggacttagggagaagggggctcaatacgggcccgaaac

SEQ ID NO: 15476 - RNA, 8669 nt, Homo sapiens
  source 1..8669: mol_type = other RNA
gctgggattacaggcatgagccactgtaccaggctgagtccacacttctaagcttgctgttgctctcagacttgcagaacaacctattaaacagaagtaggtaaaagttgagaaagggaagtggccaccacagaaccagttctgctgagaacgaggactcgagtcaggctatgctaccctccttccatggccatgggaaaaaggggtgtgtgctgttggtgtgagagatctggatcttaacagatcagacttaaactaatttgcccatgatgaccgtgtggatttggagggacctgggaatctcacagacctatgggatgtcccagtgatatgtcctgggcttcataccagccctgccctgcctgacaagttggatgaaaactgataaaggacttgtcatagcttcagatggcaaaaccaggccaggccagaatgaaaaaggagaaggaatttaacatgggcaaatgccaagctctgcatttaactaaccaaggctgcttggcgtgaacaaaactgagacagagcaatgcatggagaaaagggttgggcatttgtgggctacaagcttggcatgacatggatgcaaatgtcaatgggtgcacccccagatgcctgtgactccctctggtggtttctgtgcacaacttcccccaaaataggccctacgactccagcagaaacctaccctggggctcctagagcttcctagcctgcctgccagagagcagaagtgcctggaggctacatcttcacccctgggtagtccttactctgaggtgggactgcatccagggctcccctttagggtctgacttggactgaaatcacaccctgccttgccttctgcccctcccttaacttgctctcccctccctaataactccagcatcctcatctcagcagaagcttctggggaacccagcccaagatgagtggtgagggctagggtagccctcctcaatgcactctgggaactacattttcagaagccccagccagagggccaagtcccaggcagggtgcaaagctgtggggcgaggaacctggaaagaggctctgaacaagggacttttaaggaagtgggatgtgggctgtgatcacagccaagctggcagggtaagaggtggcccctgaatgtggctatgagaggggtgcccaacactaccagcctgtgtgctgagcactaactcagtgccaggcactacttgggttattctatttaatctccacaccaagcatgtgaaggaggcaccattgtcatccccatcttacagatgaggaagatgatcaaggcttgtaacttgcccaagatcacatggctataggtgtggatcctatatatccagattcaaactccagctttagcccactaagctacggtggccaaccccagcccaaagtgttgggacctgcgtgtagaagaccccttcagcccttgtaaagttaggatctagcatgtctaaggggacagagacccaatccaggtgacacaggaggtaagatcacagtggaacaggccatccctgcttttccaccaccaccagcactgtgacctcagaccagctctactctatgagtttcttgtgacagtgatggcagcctggggccagacaagggatgcgtgtcttgtgtcctggacacaagacaggcaggcccagaggggacaagctatatgaagagaggcttcagctgtcgggggtcctgaatgccatggaaggagagcaggtgggcagaagcagggagcccctggagcagacagaggggggattcctgctgaggcaaggggctctaggactccagggtttatgctccaaagaacagaatttaccaggacaaaataaacaagaccagtcaggaccgatgccccatccctgctggggtctggcaaagctctcacctccaaatttgtatctgttttgaattcaaagccaaacaaacacatcaacagtgaactccaacacctcccagagcagggcctgaaagggacccagaaagtctggccagaaatctagagtccaaggggaggagatctgtaaactaaaccgctggccatgctctggggccctaaaccactgcaggcatcagggctgttccaggagagggcacagcaaagggggttgggaggggtctccagttccaatcagaaatgaggctgcagtcacttcaggtagacctgtcagcagcagctgtgcaactgggctagggagacaaggatcgtggtttagccaggagaatcatctggggccccagccaagacacaggtgttggatttcagcaccgctctgcaaatactcatctcagtgacgatgaggtgagtgggagcttggctgagcccagcccggcctgccatcctggcaagccagggcagcatggaggtagcacagagtggcacccagccagcgtgaatgcataagaatctgcacgtgacacagaagaaagtctcttcatgaagtaggtttcactggtcccagccaaaccctgtggcaggtggccctttctgcacctgctgaacatgccattcaccttgacccaggtagtggcctcaccctcctcttgctcaaactggaaacctcagcatcctgaaatgcctcctccccaaatccattgcacacatgtgtgcctgtgtatgcgtgtgtgtgcacgtgtatgaacccagcccccagctgcccactccattgcccctaaacaggcccctccttggtgtcacctggcacatctccactggaagccaaatggatatttctaaactgaaatctggtcccacctcagaaccccttccacagttcccttaaagttcctttcctcatttacatcaggatcttcacaatggggacccctggtcacctcccaacccaacaaacgctccaaatgagccgccactgcagaaactcattatggcccaggcaggacaggcacatccaagtatctgaccaggctgttccatctgccaggcaggtcctgccctctctccacccacctgtctaacccctgcatcctcaagaccctacttagctatggccctgtgtgaaaggtccctccccatgcacccacagccatttgttctctctcatgtggccctaacaggctggggttcctggagactccatggggagccaggcatgaagatggcatatacccatgtgtcactccccagaacgtgagctgcctgccctggcaccatacacaaagggactgacagccccagaatcccaaggggtgcacctatgcatatgggaaaggcatgtttacgggtgagaatggtccatcgttgggcttcaggaggcatctgacctgacgcacgcctttgtcactttgtccttgtggcctgttgaaatgccactcctgctttacaaattcaccaactgttgcatgagtcatttccacctcaatgagtaccaggtccttgaggatggggaaaagtaagccaccactgtgggggtcctgggctcctaggtgcagaagaggctccagaaacaggccaggtcgtgggccatgaccccacactagccctctggtccctcacacgggtggattggggggctgtgtcacgggatcttaggatcttcaagacaaagacccaggacaagaacacaagcccactcccattcttcacaggcctcgagaaatctttgggcaatgaagtcagactgtgccaaagcccatgtttctgtctctccaaggcccctggcccccactgcctagcctaggtcaggtcatgtgggcaagcgagcccccacagcctcacagcccctaccccagggccagggcaaactcctgccctgtccccctccattcctgccctccctccttccacaaactgcaccagctggggagaaatccttcagccgacagaatgaggtgaaaatagtgcaattttaggctttgtaactgagattagggcaggtggccacccattctccccttcctcaggccagcctctgacacaatgaccctggaagcctggcagccctccgtaatggtcagcatcctcccctgccatccccaacccacaccatgagctcagccagggcaggggcagcctctgtctcattcaccacagaatccacagaacccagcacagagtatgagctcagtaaattctcctcatacatgactgcactgactggaccgggcacatgctacagggcaacacccacggctcagctggccctggctttggatctcagtcccacctcttcaagctgtccagcgtggggcacatcggctacagccttgccaaatgaaggcttgccaggatgaagaggtgaagacaggacaagcacagtatgtggcacacaggaggcctctgataacatcagtccccttccctaaagacctgggcagtccctgtcactggggcctcacatttcatgtcgagaattcactatttctcagcactgatttcaaataaagccaccaagagtctgacgaggcaacatggcagagttctgagggtggagtgaacaaaaggtcattttttacagaaaactcaggatctcccctctgcacagtgctaaagccctgtctcaaagttcagagcccggaaggtgcagagatgtggcccttggaaatcaagcccttaagaaaacagcccagctgtgtagggccggaagccccaggctgcagtcctgtggtctggaggcagccaatattcaggtgagagatgtgcccagctgccggtgggtccagggggcacggagcccccaccgtccctggcccaggtctaggactaagtcagtgggcccaggccagctccaagggccacagctcctcactcgggggccgcgccggagcagccgcagcagctggggcgccgcagggactgcatgacagcccgcagtggccccctccggccctccacagacaggctgtcctcgctggcgggcgcccgctgcagctgctcaaactgcatctccaggtgcttctggatggccacaccgagcacctccaggtccaccgcagctccgtacacctcccatgtcatgccctcagcatcccatcgcacatcccgcacaggggacggcacctcctccaggctggaccccagagttacctctgggaacacatgcagggctgcaggcgcttccagggacggactggtggccacagccttgcaggccgccactggggccgcctgcacaccagcatcctgggctgacagcggggatgcctctgcaggggccaagtcattggctgaggtcatggtccacacatctttggtcctagagccaggctctgggactaacccagcgggaccccaaaggtgggcacagcaatgggaatgcccagggagccccccagacaacctacagtggatcttcaccccatgctgagcctgcagcccagactcgctcactgacgccactagtttgggaaaggccaggatccctgtggcaggtagggcatggcagcagccaccagccctcacctccctcatgccacagagtagagcagctgggggcagagcatggcaggtggtggtagccagctgttcagcagctttgggctcagcctgggcactgctgctgtgggcagttgtgtcccccaggtctagtggtggcactgacaactgactcgcccccagcatccaggctgagttagaagtctcatcctcaggagccaggtccctttccaggcctgcaggggcctggccaccctggccagaagtaccacctggctgcagctgagccctgtggacagggctgctgccaagggctgagcagctgagactggccttccgagcaccactgtgtccccgcatctgggtgctacggaccaggtctgaatggctcctctgcatagcagcagcactaggggcccgcaggcgacacaggtcactgccgcccatggtggacacattgcccacagtgctgctccaccagtggcctccagcactgggtcgcgccttggggccagaggcccgtgctggcttcatgctctcaggcgggttcccctcttcctccggggcctggggtctggtgctggcctcgcccagctgggcctgccacacggtgctgctggcagtcttgcggagctctggcctctgttcccggccttcacccagcaggctggaagagctctgggacaggggctgaaggcgggggctcaggggtgcccagggacccggctcggggcggctggagctcatggctgcctctagctccaggggcaaggagaggccccatgcatcagctttttccatgagggactcattcagcatctggtcattgattccacagcatctcctgagcccctactgcgtgcccagctgtagggctagggaacatgggattcattcagacctttctgtacccctgatgtgtcgtcggcactcagaggattatctgctgtgtgcctgaccaagagaacaagcaaatacaagaacacacccacagaggagggcactgagtgccaaaaatggggtctgagggagggcaccaccaaggcaggagagctcacggagggtgagagatgagaaaaggcttcctggaggaccagccacgtaagtcaggcctggagtgagagaagcaagaaggtgttcaggtggagagcggagtgggcaggaggaaagaggccatgtgtccagagcatatgaggggagcagtggggtcaaagtgtctgggccacctcggccctggccacagcagtgaattagggagatcactctgggactccttgccaggcaggagaggtgggagaaacagggtggggacaggaggcagcagctgcatttgggcaatcccagccctgccctcccagcctaggctgataaagacttccaggcaacaacctccccgaccaggtgagcaaggctacccgagaggaaattcgggaagggctgtgggactcggtttctgtgtaattacaaatgtcctggcagcccagcactcaggagatggctggtggctgctgagccacagtgaggatgatactggtgctgtagtccctgagactccagctctgcacaacttcctgcgatgatggaaagattctaccctgtgctgtccaataggtaggcaccaatggcatgtgggtaccaagcactcagcagggggctactgcaactgagacactgaatgtttaagttttatttgaatctaactggccacatgaggctaatggctaccgtacaggactgtgcagctctgaacacagccccggcctggtaaggatgtcccatcccagctgcttcacggggctgaagccagacttgtccctgggaggatcaggaagaggaggagtagccaagagagaaatctgacccagaccctgccctcaatgagctctaagatggacatacaaacaaaggagggcaataaagcccgtaacagcgatgataataacagctgccagggcctgatcactcgccaagggccagacacgtgccacatcctttgcatacattgtctcatataactgtgcaagcaacctcttgagacagtcattatctccattctacagacaggagaattccataagctcagagaggctcagtgacccccaagggcacacacctgtggggcagctgagctcctctccccttcgagcactgagcaggcctatgcctcgcagctctcaccctttttactgatctggcctggccctgccaatcgtgctcatgacatgccatggaacaagtcactgagtggatctccacctgcccaacatgcttcttagcagctcctgaggctgcaagaatgaggagggcaggaggtgttcctcctgactgggacagctgtggtcactgccagcccctggcagggagacaaccactcagttgcaggtccaagaccccagggaggccccatctggacatccacacagcctctggccaaaccccaccaccctcccagggaggggggccataaacagccaggccagcagcctctggcccctgaggagacaggtggaatgaggtcctcagacccccaccaagacccactgagaagccatgagcaatgagcatcccactgtgcctgtctcaccagagggctgcccagcacccagggctagtcatcacccagagacccccgtgtgggctatgtatctattggttcccttccccattccccctccacaagtggcaggtgacaaaactgaggcctggagcagctcagaaatgtcaaagaacacacagctgaaagtggctaattcagaaccccaatggattggcctggctaactacaacctggccttcccagctcagaaggaaggaagggctctgaggggagtactgggggaaagaggcttccacactgcctgtcacagtgctgtggactgggccagaggaggggcctcccagggagccaggggtgaggaggaaggggcagggctctgcttccaatgggggctcttccccttcctgtgcatgtactcacaggtggacccctaacttctttgagcctcagtttcttcaatcttaatgttctctctcctgccccatttgatgccgaagttgctatggttgtggccgatgtcccgtggccaatgccaggctgtcctgctgcctcaggttccacctgtcagcaacctctcgcccgccggggccgcgcaggcgggggaagcgctgctcctgcggccgccacaggtgccaggtgccgcggcccaagatggagccagagccgacctggcctgggcgcgagacgccgcccgccgccgtcggcccggcc

SEQ ID NO: 15477 - RNA, 8824 nt, Homo sapiens
  source 1..8824: mol_type = other RNA
gctgggattacaggcatgagccactgtaccaggctgagtccacacttctaagcttgctgttgctctcagacttgcagaacaacctattaaacagaagtaggtaaaagttgagaaagggaagtggccaccacagaaccagttctgctgagaacgaggactcgagtcaggctatgctaccctccttccatggccatgggaaaaaggggtgtgtgctgttggtgtgagagatctggatcttaacagatcagacttaaactaatttgcccatgatgaccgtgtggatttggagggacctgggaatctcacagacctatgggatgtcccagtgatatgtcctgggcttcataccagccctgccctgcctgacaagttggatgaaaactgataaaggacttgtcatagcttcagatggcaaaaccaggccaggccagaatgaaaaaggagaaggaatttaacatgggcaaatgccaagctctgcatttaactaaccaaggctgcttggcgtgaacaaaactgagacagagcaatgcatggagaaaagggttgggcatttgtgggctacaagcttggcatgacatggatgcaaatgtcaatgggtgcacccccagatgcctgtgactccctctggtggtttctgtgcacaacttcccccaaaataggccctacgactccagcagaaacctaccctggggctcctagagcttcctagcctgcctgccagagagcagaagtgcctggaggctacatcttcacccctgggtagtccttactctgaggtgggactgcatccagggctcccctttagggtctgacttggactgaaatcacaccctgccttgccttctgcccctcccttaacttgctctcccctccctaataactccagcatcctcatctcagcagaagcttctggggaacccagcccaagatgagtggtgagggctagggtagccctcctcaatgcactctgggaactacattttcagaagccccagccagagggccaagtcccaggcagggtgcaaagctgtggggcgaggaacctggaaagaggctctgaacaagggacttttaaggaagtgggatgtgggctgtgatcacagccaagctggcagggtaagaggtggcccctgaatgtggctatgagaggggtgcccaacactaccagcctgtgtgctgagcactaactcagtgccaggcactacttgggttattctatttaatctccacaccaagcatgtgaaggaggcaccattgtcatccccatcttacagatgaggaagatgatcaaggcttgtaacttgcccaagatcacatggctataggtgtggatcctatatatccagattcaaactccagctttagcccactaagctacggtggccaaccccagcccaaagtgttgggacctgcgtgtagaagaccccttcagcccttgtaaagttaggatctagcatgtctaaggggacagagacccaatccaggtgacacaggaggtaagatcacagtggaacaggccatccctgcttttccaccaccaccagcactgtgacctcagaccagctctactctatgagtttcttgtgacagtgatggcagcctggggccagacaagggatgcgtgtcttgtgtcctggacacaagacaggcaggcccagaggggacaagctatatgaagagaggcttcagctgtcgggggtcctgaatgccatggaaggagagcaggtgggcagaagcagggagcccctggagcagacagaggggggattcctgctgaggcaaggggctctaggactccagggtttatgctccaaagaacagaatttaccaggacaaaataaacaagaccagtcaggaccgatgccccatccctgctggggtctggcaaagctctcacctccaaatttgtatctgttttgaattcaaagccaaacaaacacatcaacagtgaactccaacacctcccagagcagggcctgaaagggacccagaaagtctggccagaaatctagagtccaaggggaggagatctgtaaactaaaccgctggccatgctctggggccctaaaccactgcaggcatcagggctgttccaggagagggcacagcaaagggggttgggaggggtctccagttccaatcagaaatgaggctgcagtcacttcaggtagacctgtcagcagcagctgtgcaactgggctagggagacaaggatcgtggtttagccaggagaatcatctggggccccagccaagacacaggtgttggatttcagcaccgctctgcaaatactcatctcagtgacgatgaggtgagtgggagcttggctgagcccagcccggcctgccatcctggcaagccagggcagcatggaggtagcacagagtggcacccagccagcgtgaatgcataagaatctgcacgtgacacagaagaaagtctcttcatgaagtaggtttcactggtcccagccaaaccctgtggcaggtggccctttctgcacctgctgaacatgccattcaccttgacccaggtagtggcctcaccctcctcttgctcaaactggaaacctcagcatcctgaaatgcctcctccccaaatccattgcacacatgtgtgcctgtgtatgcgtgtgtgtgcacgtgtatgaacccagcccccagctgcccactccattgcccctaaacaggcccctccttggtgtcacctggcacatctccactggaagccaaatggatatttctaaactgaaatctggtcccacctcagaaccccttccacagttcccttaaagttcctttcctcatttacatcaggatcttcacaatggggacccctggtcacctcccaacccaacaaacgctccaaatgagccgccactgcagaaactcattatggcccaggcaggacaggcacatccaagtatctgaccaggctgttccatctgccaggcaggtcctgccctctctccacccacctgtctaacccctgcatcctcaagaccctacttagctatggccctgtgtgaaaggtccctccccatgcacccacagccatttgttctctctcatgtggccctaacaggctggggttcctggagactccatggggagccaggcatgaagatggcatatacccatgtgtcactccccagaacgtgagctgcctgccctggcaccatacacaaagggactgacagccccagaatcccaaggggtgcacctatgcatatgggaaaggcatgtttacgggtgagaatggtccatcgttgggcttcaggaggcatctgacctgacgcacgcctttgtcactttgtccttgtggcctgttgaaatgccactcctgctttacaaattcaccaactgttgcatgagtcatttccacctcaatgagtaccaggtccttgaggatggggaaaagtaagccaccactgtgggggtcctgggctcctaggtgcagaagaggctccagaaacaggccaggtcgtgggccatgaccccacactagccctctggtccctcacacgggtggattggggggctgtgtcacgggatcttaggatcttcaagacaaagacccaggacaagaacacaagcccactcccattcttcacaggcctcgagaaatctttgggcaatgaagtcagactgtgccaaagcccatgtttctgtctctccaaggcccctggcccccactgcctagcctaggtcaggtcatgtgggcaagcgagcccccacagcctcacagcccctaccccagggccagggcaaactcctgccctgtccccctccattcctgccctccctccttccacaaactgcaccagctggggagaaatccttcagccgacagaatgaggtgaaaatagtgcaattttaggctttgtaactgagattagggcaggtggccacccattctccccttcctcaggccagcctctgacacaatgaccctggaagcctggcagccctccgtaatggtcagcatcctcccctgccatccccaacccacaccatgagctcagccagggcaggggcagcctctgtctcattcaccacagaatccacagaacccagcacagagtatgagctcagtaaattctcctcatacatgactgcactgactggaccgggcacatgctacagggcaacacccacggctcagctggccctggctttggatctcagtcccacctcttcaagctgtccagcgtggggcacatcggctacagccttgccaaatgaaggcttgccaggatgaagaggtgaagacaggacaagcacagtatgtggcacacaggaggcctctgataacatcagtccccttccctaaagacctgggcagtccctgtcactggggcctcacatttcatgtcgagaattcactatttctcagcactgatttcaaataaagccaccaagagtctgacgaggcaacatggcagagttctgagggtggagtgaacaaaaggtcattttttacagaaaactcaggatctcccctctgcacagtgctaaagccctgtctcaaagttcagagcccggaaggtgcagagatgtggcccttggaaatcaagcccttaagaaaacagcccagctgtgtagggccggaagccccaggctgcagtcctgtggtctggaggcagccaatattcaggtgagagatgtgcccagctgccggtgggtccagggggcacggagcccccaccgtccctggcccaggtctaggactaagtcagtgggcccaggccagctccaagggccacagctcctcactcgggggccgcgccggagcagccgcagcagctggggcgccgcagggactgcatgacagcccgcagtggccccctccggccctccacagacaggctgtcctcgctggcgggcgcccgctgcagctgctcaaactgcatctccaggtgcttctggatggccacaccgagcacctccaggtccaccgcagctccgtacacctcccatgtcatgccctcagcatcccatcgcacatcccgcacaggggacggcacctcctccaggctggaccccagagttacctctgggaacacatgcagggctgcaggcgcttccagggacggactggtggccacagccttgcaggccgccactggggccgcctgcacaccagcatcctgggctgacagcggggatgcctctgcaggggccaagtcattggctgaggtcatggtccacacatctttggtcctagagccaggctctgggactaacccagcgggaccccaaaggtgggcacagcaatgggaatgcccagggagccccccagacaacctacagtggatcttcaccccatgctgagcctgcagcccagactcgctcactgacgccactagtttgggaaaggccaggatccctgtggcaggtagggcatggcagcagccaccagccctcacctccctcatgccacagagtagagcagctgggggcagagcatggcaggtggtggtagccagctgttcagcagctttgggctcagcctgggcactgctgctgtgggcagttgtgtcccccaggtctagtggtggcactgacaactgactcgcccccagcatccaggctgagttagaagtctcatcctcaggagccaggtccctttccaggcctgcaggggcctggccaccctggccagaagtaccacctggctgcagctgagccctgtggacagggctgctgccaagggctgagcagctgagactggccttccgagcaccactgtgtccccgcatctgggtgctacggaccaggtctgaatggctcctctgcatagcagcagcactaggggcccgcaggcgacacaggtcactgccgcccatggtggacacattgcccacagtgctgctccaccagtggcctccagcactgggtcgcgccttggggccagaggcccgtgctggcttcatgctctcaggcgggttcccctcttcctccggggcctggggtctggtgctggcctcgcccagctgggcctgccacacggtgctgctggcagtcttgcggagctctggcctctgttcccggccttcacccagcaggctggaagagctctgggacaggggctgaaggcgggggctcaggggtgcccagggacccggctcggggcggctggagctcatggctgcctctagctccaggggcaaggagaggccccatgcatcagctttttccatgagggactcattcagcatctggtcattgattccacagcatctcctgagcccctactgcgtgcccagctgtagggctagggaacatgggattcattcagacctttctgtacccctgatgtgtcgtcggcactcagaggattatctgctgtgtgcctgaccaagagaacaagcaaatacaagaacacacccacagaggagggcactgagtgccaaaaatggggtctgagggagggcaccaccaaggcaggagagctcacggagggtgagagatgagaaaaggcttcctggaggaccagccacgtaagtcaggcctggagtgagagaagcaagaaggtgttcaggtggagagcggagtgggcaggaggaaagaggccatgtgtccagagcatatgaggggagcagtggggtcaaagtgtctgggccacctcggccctggccacagcagtgaattagggagatcactctgggactccttgccaggcaggagaggtgggagaaacagggtggggacaggaggcagcagctgcatttgggcaatcccagccctgccctcccagcctaggctgataaagacttccaggcaacaacctccccgaccaggtgagcaaggctacccgagaggaaattcgggaagggctgtgggactcggtttctgtgtaattacaaatgtcctggcagcccagcactcaggagatggctggtggctgctgagccacagtgaggatgatactggtgctgtagtccctgagactccagctctgcacaacttcctgcgatgatggaaagattctaccctgtgctgtccaataggtaggcaccaatggcatgtgggtaccaagcactcagcagggggctactgcaactgagacactgaatgtttaagttttatttgaatctaactggccacatgaggctaatggctaccgtacaggactgtgcagctctgaacacagccccggcctggtaaggatgtcccatcccagctgcttcacggggctgaagccagacttgtccctgggaggatcaggaagaggaggagtagccaagagagaaatctgacccagaccctgccctcaatgagctctaagatggacatacaaacaaaggagggcaataaagcccgtaacagcgatgataataacagctgccagggcctgatcactcgccaagggccagacacgtgccacatcctttgcatacattgtctcatataactgtgcaagcaacctcttgagacagtcattatctccattctacagacaggagaattccataagctcagagaggctcagtgacccccaagggcacacacctgtggggcagctgagctcctctccccttcgagcactgagcaggcctatgcctcgcagctctcaccctttttactgatctggcctggccctgccaatcgtgctcatgacatgccatggaacaagtcactgagtggatctccacctgcccaacatgcttcttagcagctcctgaggctgcaagaatgaggagggcaggaggtgttcctcctgactgggacagctgtggtcactgccagcccctggcagggagacaaccactcagttgcaggtccaagaccccagggaggccccatctggacatccacacagcctctggccaaaccccaccaccctcccagggaggggggccataaacagccaggccagcagcctctggcccctgaggagacaggtggaatgaggtcctcagacccccaccaagacccactgagaagccatgagcaatgagcatcccactgtgcctgtctcaccagagggctgcccagcacccagggctagtcatcacccagagacccccgtgtgggctatgtatctattggttcccttccccattccccctccacaagtggcaggtgacaaaactgaggcctggagcagctcagaaatgtcaaagaacacacagctgaaagtggctaattcagaaccccaatggattggcctggctaactacaacctggccttcccagctcagaaggaaggaagggctctgaggggagtactgggggaaagaggcttccacactgcctgtcacagtgctgtggactgggccagaggaggggcctcccagggagccaggggtgaggaggaaggggcagggctctgcttccaatgggggctcttccccttcctgtgcatgtactcacaggtggacccctaacttctttgagcctcagtttcttcaatcttaatgttctctctcctgccccatttgatgccgaagttgctatggttgtggccgatgtcccgtggccaatgccaggctgtcctgctgcctcaggttccacctgtcagcaactctcaaggaccaggcaggaatgcacacagcacaaacccccattgcacagtggggatacagcaccctccaggaggtggtttaatccaccccagagtgaacggggcctgataggaacactcagggccaactctgggcaaagcagcaggcagcattccctctcgcccgccggggccgcgcaggcgggggaagcgctgctcctgcggccgccacaggtgccaggtgccgcggcccaagatggagccagagccgacctggcctgggcgcgagacgccgcccgccgccgtcggcccggcc

SEQ ID NO: 15478 - RNA, 9099 nt, Homo sapiens
  source 1..9099: mol_type = other RNA
gctgggattacaggcatgagccactgtaccaggctgagtccacacttctaagcttgctgttgctctcagacttgcagaacaacctattaaacagaagtaggtaaaagttgagaaagggaagtggccaccacagaaccagttctgctgagaacgaggactcgagtcaggctatgctaccctccttccatggccatgggaaaaaggggtgtgtgctgttggtgtgagagatctggatcttaacagatcagacttaaactaatttgcccatgatgaccgtgtggatttggagggacctgggaatctcacagacctatgggatgtcccagtgatatgtcctgggcttcataccagccctgccctgcctgacaagttggatgaaaactgataaaggacttgtcatagcttcagatggcaaaaccaggccaggccagaatgaaaaaggagaaggaatttaacatgggcaaatgccaagctctgcatttaactaaccaaggctgcttggcgtgaacaaaactgagacagagcaatgcatggagaaaagggttgggcatttgtgggctacaagcttggcatgacatggatgcaaatgtcaatgggtgcacccccagatgcctgtgactccctctggtggtttctgtgcacaacttcccccaaaataggccctacgactccagcagaaacctaccctggggctcctagagcttcctagcctgcctgccagagagcagaagtgcctggaggctacatcttcacccctgggtagtccttactctgaggtgggactgcatccagggctcccctttagggtctgacttggactgaaatcacaccctgccttgccttctgcccctcccttaacttgctctcccctccctaataactccagcatcctcatctcagcagaagcttctggggaacccagcccaagatgagtggtgagggctagggtagccctcctcaatgcactctgggaactacattttcagaagccccagccagagggccaagtcccaggcagggtgcaaagctgtggggcgaggaacctggaaagaggctctgaacaagggacttttaaggaagtgggatgtgggctgtgatcacagccaagctggcagggtaagaggtggcccctgaatgtggctatgagaggggtgcccaacactaccagcctgtgtgctgagcactaactcagtgccaggcactacttgggttattctatttaatctccacaccaagcatgtgaaggaggcaccattgtcatccccatcttacagatgaggaagatgatcaaggcttgtaacttgcccaagatcacatggctataggtgtggatcctatatatccagattcaaactccagctttagcccactaagctacggtggccaaccccagcccaaagtgttgggacctgcgtgtagaagaccccttcagcccttgtaaagttaggatctagcatgtctaaggggacagagacccaatccaggtgacacaggaggtaagatcacagtggaacaggccatccctgcttttccaccaccaccagcactgtgacctcagaccagctctactctatgagtttcttgtgacagtgatggcagcctggggccagacaagggatgcgtgtcttgtgtcctggacacaagacaggcaggcccagaggggacaagctatatgaagagaggcttcagctgtcgggggtcctgaatgccatggaaggagagcaggtgggcagaagcagggagcccctggagcagacagaggggggattcctgctgaggcaaggggctctaggactccagggtttatgctccaaagaacagaatttaccaggacaaaataaacaagaccagtcaggaccgatgccccatccctgctggggtctggcaaagctctcacctccaaatttgtatctgttttgaattcaaagccaaacaaacacatcaacagtgaactccaacacctcccagagcagggcctgaaagggacccagaaagtctggccagaaatctagagtccaaggggaggagatctgtaaactaaaccgctggccatgctctggggccctaaaccactgcaggcatcagggctgttccaggagagggcacagcaaagggggttgggaggggtctccagttccaatcagaaatgaggctgcagtcacttcaggtagacctgtcagcagcagctgtgcaactgggctagggagacaaggatcgtggtttagccaggagaatcatctggggccccagccaagacacaggtgttggatttcagcaccgctctgcaaatactcatctcagtgacgatgaggtgagtgggagcttggctgagcccagcccggcctgccatcctggcaagccagggcagcatggaggtagcacagagtggcacccagccagcgtgaatgcataagaatctgcacgtgacacagaagaaagtctcttcatgaagtaggtttcactggtcccagccaaaccctgtggcaggtggccctttctgcacctgctgaacatgccattcaccttgacccaggtagtggcctcaccctcctcttgctcaaactggaaacctcagcatcctgaaatgcctcctccccaaatccattgcacacatgtgtgcctgtgtatgcgtgtgtgtgcacgtgtatgaacccagcccccagctgcccactccattgcccctaaacaggcccctccttggtgtcacctggcacatctccactggaagccaaatggatatttctaaactgaaatctggtcccacctcagaaccccttccacagttcccttaaagttcctttcctcatttacatcaggatcttcacaatggggacccctggtcacctcccaacccaacaaacgctccaaatgagccgccactgcagaaactcattatggcccaggcaggacaggcacatccaagtatctgaccaggctgttccatctgccaggcaggtcctgccctctctccacccacctgtctaacccctgcatcctcaagaccctacttagctatggccctgtgtgaaaggtccctccccatgcacccacagccatttgttctctctcatgtggccctaacaggctggggttcctggagactccatggggagccaggcatgaagatggcatatacccatgtgtcactccccagaacgtgagctgcctgccctggcaccatacacaaagggactgacagccccagaatcccaaggggtgcacctatgcatatgggaaaggcatgtttacgggtgagaatggtccatcgttgggcttcaggaggcatctgacctgacgcacgcctttgtcactttgtccttgtggcctgttgaaatgccactcctgctttacaaattcaccaactgttgcatgagtcatttccacctcaatgagtaccaggtccttgaggatggggaaaagtaagccaccactgtgggggtcctgggctcctaggtgcagaagaggctccagaaacaggccaggtcgtgggccatgaccccacactagccctctggtccctcacacgggtggattggggggctgtgtcacgggatcttaggatcttcaagacaaagacccaggacaagaacacaagcccactcccattcttcacaggcctcgagaaatctttgggcaatgaagtcagactgtgccaaagcccatgtttctgtctctccaaggcccctggcccccactgcctagcctaggtcaggtcatgtgggcaagcgagcccccacagcctcacagcccctaccccagggccagggcaaactcctgccctgtccccctccattcctgccctccctccttccacaaactgcaccagctggggagaaatccttcagccgacagaatgaggtgaaaatagtgcaattttaggctttgtaactgagattagggcaggtggccacccattctccccttcctcaggccagcctctgacacaatgaccctggaagcctggcagccctccgtaatggtcagcatcctcccctgccatccccaacccacaccatgagctcagccagggcaggggcagcctctgtctcattcaccacagaatccacagaacccagcacagagtatgagctcagtaaattctcctcatacatgactgcactgactggaccgggcacatgctacagggcaacacccacggctcagctggccctggctttggatctcagtcccacctcttcaagctgtccagcgtggggcacatcggctacagccttgccaaatgaaggcttgccaggatgaagaggtgaagacaggacaagcacagtatgtggcacacaggaggcctctgataacatcagtccccttccctaaagacctgggcagtccctgtcactggggcctcacatttcatgtcgagaattcactatttctcagcactgatttcaaataaagccaccaagagtctgacgaggcaacatggcagagttctgagggtggagtgaacaaaaggtcattttttacagaaaactcaggatctcccctctgcacagtgctaaagccctgtctcaaagttcagagcccggaaggtgcagagatgtggcccttggaaatcaagcccttaagaaaacagcccagctgtgtagggccggaagccccaggctgcagtcctgtggtctggaggcagccaatattcaggtgagagatgtgcccagctgccggtgggtccagggggcacggagcccccaccgtccctggcccaggtctaggactaagtcagtgggcccaggccagctccaagggccacagctcctcactcgggggccgcgccggagcagccgcagcagctggggcgccgcagggactgcatgacagcccgcagtggccccctccggccctccacagacaggctgtcctcgctggcgggcgcccgctgcagctgctcaaactgcatctccaggtgcttctggatggccacaccgagcacctccaggtccaccgcagctccgtacacctcccatgtcatgccctcagcatcccatcgcacatcccgcacaggggacggcacctcctccaggctggaccccagagttacctctgggaacacatgcagggctgcaggcgcttccagggacggactggtggccacagccttgcaggccgccactggggccgcctgcacaccagcatcctgggctgacagcggggatgcctctgcaggggccaagtcattggctgaggtcatggtccacacatctttggtcctagagccaggctctgggactaacccagcgggaccccaaaggtgggcacagcaatgggaatgcccagggagccccccagacaacctacagtggatcttcaccccatgctgagcctgcagcccagactcgctcactgacgccactagtttgggaaaggccaggatccctgtggcaggtagggcatggcagcagccaccagccctcacctccctcatgccacagagtagagcagctgggggcagagcatggcaggtggtggtagccagctgttcagcagctttgggctcagcctgggcactgctgctgtgggcagttgtgtcccccaggtctagtggtggcactgacaactgactcgcccccagcatccaggctgagttagaagtctcatcctcaggagccaggtccctttccaggcctgcaggggcctggccaccctggccagaagtaccacctggctgcagctgagccctgtggacagggctgctgccaagggctgagcagctgagactggccttccgagcaccactgtgtccccgcatctgggtgctacggaccaggtctgaatggctcctctgcatagcagcagcactaggggcccgcaggcgacacaggtcactgccgcccatggtggacacattgcccacagtgctgctccaccagtggcctccagcactgggtcgcgccttggggccagaggcccgtgctggcttcatgctctcaggcgggttcccctcttcctccggggcctggggtctggtgctggcctcgcccagctgggcctgccacacggtgctgctggcagtcttgcggagctctggcctctgttcccggccttcacccagcaggctggaagagctctgggacaggggctgaaggcgggggctcaggggtgcccagggacccggctcggggcggctggagctcatggctgcctctagctccaggggcaaggagaggccccatgcatcagctttttccatgagggactcattcagcatctggtcattgattccacagcatctcctgagcccctactgcgtgcccagctgtagggctagggaacatgggattcattcagacctttctgtacccctgatgtgtcgtcggcactcagaggattatctgctgtgtgcctgaccaagagaacaagcaaatacaagaacacacccacagaggagggcactgagtgccaaaaatggggtctgagggagggcaccaccaaggcaggagagctcacggagggtgagagatgagaaaaggcttcctggaggaccagccacgtaagtcaggcctggagtgagagaagcaagaaggtgttcaggtggagagcggagtgggcaggaggaaagaggccatgtgtccagagcatatgaggggagcagtggggtcaaagtgtctgggccacctcggccctggccacagcagtgaattagggagatcactctgggactccttgccaggcaggagaggtgggagaaacagggtggggacaggaggcagcagctgcatttgggcaatcccagccctgccctcccagcctaggctgataaagacttccaggcaacaacctccccgaccaggtgagcaaggctacccgagaggaaattcgggaagggctgtgggactcggtttctgtgtaattacaaatgtcctggcagcccagcactcaggagatggctggtggctgctgagccacagtgaggatgatactggtgctgtagtccctgagactccagctctgcacaacttcctgcgatgatggaaagattctaccctgtgctgtccaataggtaggcaccaatggcatgtgggtaccaagcactcagcagggggctactgcaactgagacactgaatgtttaagttttatttgaatctaactggccacatgaggctaatggctaccgtacaggactgtgcagctctgaacacagccccggcctggtaaggatgtcccatcccagctgcttcacggggctgaagccagacttgtccctgggaggatcaggaagaggaggagtagccaagagagaaatctgacccagaccctgccctcaatgagctctaagatggacatacaaacaaaggagggcaataaagcccgtaacagcgatgataataacagctgccagggcctgatcactcgccaagggccagacacgtgccacatcctttgcatacattgtctcatataactgtgcaagcaacctcttgagacagtcattatctccattctacagacaggagaattccataagctcagagaggctcagtgacccccaagggcacacacctgtggggcagctgagctcctctccccttcgagcactgagcaggcctatgcctcgcagctctcaccctttttactgatctggcctggccctgccaatcgtgctcatgacatgccatggaacaagtcactgagtggatctccacctgcccaacatgcttcttagcagctcctgaggctgcaagaatgaggagggcaggaggtgttcctcctgactgggacagctgtggtcactgccagcccctggcagggagacaaccactcagttgcaggtccaagaccccagggaggccccatctggacatccacacagcctctggccaaaccccaccaccctcccagggaggggggccataaacagccaggccagcagcctctggcccctgaggagacaggtggaatgaggtcctcagacccccaccaagacccactgagaagccatgagcaatgagcatcccactgtgcctgtctcaccagagggctgcccagcacccagggctagtcatcacccagagacccccgtgtgggctatgtatctattggttcccttccccattccccctccacaagtggcaggtgacaaaactgaggcctggagcagctcagaaatgtcaaagaacacacagctgaaagtggctaattcagaaccccaatggattggcctggctaactacaacctggccttcccagctcagaaggaaggaagggctctgaggggagtactgggggaaagaggcttccacactgcctgtcacagtgctgtggactgggccagaggaggggcctcccagggagccaggggtgaggaggaaggggcagggctctgcttccaatgggggctcttccccttcctgtgcatgtactcacaggtggacccctaacttctttgagcctcagtttcttcaatcttaatgttctctctcctgccccatttgatgccgaagttgctatggttgtggccgatgtcccgtggccaatgccaggctgtcctgctgcctcaggttccacctgtcagcaactctcaaggaccaggcaggaatgcacacagcacaaacccccattgcacagtggggatacagcaccctccaggaggtggtttaatccaccccagagtgaacggggcctgataggaacactcagggccaactctgggcaaagcagcaggcagcattccttctcaggagcaaaggcagcgactgcaggcaaatggggctgtgggccggggtaatgatgcgggacaggagaagccaaagggcagcaaggctgggggcggggtaggcggcgcagtaggctgagggaggggaaaaggaagaaggggagagggaggagcgatggcagcaggggtggaggccgaaggagacagggtcccggacagacttgtgaaaatgggaggatgggcagaggagacgtagaagaggggacaggacaggacaatgagaggcggagcgcggggagtgcgatgcggccaccgggggctctgggcgctgggcaggggccaggatgccgggggtctgagcgcaggcagcgggaaggagtgggttctgaggctcagcaagggggaggtgccgcccaccacgccccccgcccc

SEQ ID NO: 15479 - RNA, 8685 nt, Homo sapiens
  source 1..8685: mol_type = other RNA
gctgggattacaggcatgagccactgtaccaggctgagtccacacttctaagcttgctgttgctctcagacttgcagaacaacctattaaacagaagtaggtaaaagttgagaaagggaagtggccaccacagaaccagttctgctgagaacgaggactcgagtcaggctatgctaccctccttccatggccatgggaaaaaggggtgtgtgctgttggtgtgagagatctggatcttaacagatcagacttaaactaatttgcccatgatgaccgtgtggatttggagggacctgggaatctcacagacctatgggatgtcccagtgatatgtcctgggcttcataccagccctgccctgcctgacaagttggatgaaaactgataaaggacttgtcatagcttcagatggcaaaaccaggccaggccagaatgaaaaaggagaaggaatttaacatgggcaaatgccaagctctgcatttaactaaccaaggctgcttggcgtgaacaaaactgagacagagcaatgcatggagaaaagggttgggcatttgtgggctacaagcttggcatgacatggatgcaaatgtcaatgggtgcacccccagatgcctgtgactccctctggtggtttctgtgcacaacttcccccaaaataggccctacgactccagcagaaacctaccctggggctcctagagcttcctagcctgcctgccagagagcagaagtgcctggaggctacatcttcacccctgggtagtccttactctgaggtgggactgcatccagggctcccctttagggtctgacttggactgaaatcacaccctgccttgccttctgcccctcccttaacttgctctcccctccctaataactccagcatcctcatctcagcagaagcttctggggaacccagcccaagatgagtggtgagggctagggtagccctcctcaatgcactctgggaactacattttcagaagccccagccagagggccaagtcccaggcagggtgcaaagctgtggggcgaggaacctggaaagaggctctgaacaagggacttttaaggaagtgggatgtgggctgtgatcacagccaagctggcagggtaagaggtggcccctgaatgtggctatgagaggggtgcccaacactaccagcctgtgtgctgagcactaactcagtgccaggcactacttgggttattctatttaatctccacaccaagcatgtgaaggaggcaccattgtcatccccatcttacagatgaggaagatgatcaaggcttgtaacttgcccaagatcacatggctataggtgtggatcctatatatccagattcaaactccagctttagcccactaagctacggtggccaaccccagcccaaagtgttgggacctgcgtgtagaagaccccttcagcccttgtaaagttaggatctagcatgtctaaggggacagagacccaatccaggtgacacaggaggtaagatcacagtggaacaggccatccctgcttttccaccaccaccagcactgtgacctcagaccagctctactctatgagtttcttgtgacagtgatggcagcctggggccagacaagggatgcgtgtcttgtgtcctggacacaagacaggcaggcccagaggggacaagctatatgaagagaggcttcagctgtcgggggtcctgaatgccatggaaggagagcaggtgggcagaagcagggagcccctggagcagacagaggggggattcctgctgaggcaaggggctctaggactccagggtttatgctccaaagaacagaatttaccaggacaaaataaacaagaccagtcaggaccgatgccccatccctgctggggtctggcaaagctctcacctccaaatttgtatctgttttgaattcaaagccaaacaaacacatcaacagtgaactccaacacctcccagagcagggcctgaaagggacccagaaagtctggccagaaatctagagtccaaggggaggagatctgtaaactaaaccgctggccatgctctggggccctaaaccactgcaggcatcagggctgttccaggagagggcacagcaaagggggttgggaggggtctccagttccaatcagaaatgaggctgcagtcacttcaggtagacctgtcagcagcagctgtgcaactgggctagggagacaaggatcgtggtttagccaggagaatcatctggggccccagccaagacacaggtgttggatttcagcaccgctctgcaaatactcatctcagtgacgatgaggtgagtgggagcttggctgagcccagcccggcctgccatcctggcaagccagggcagcatggaggtagcacagagtggcacccagccagcgtgaatgcataagaatctgcacgtgacacagaagaaagtctcttcatgaagtaggtttcactggtcccagccaaaccctgtggcaggtggccctttctgcacctgctgaacatgccattcaccttgacccaggtagtggcctcaccctcctcttgctcaaactggaaacctcagcatcctgaaatgcctcctccccaaatccattgcacacatgtgtgcctgtgtatgcgtgtgtgtgcacgtgtatgaacccagcccccagctgcccactccattgcccctaaacaggcccctccttggtgtcacctggcacatctccactggaagccaaatggatatttctaaactgaaatctggtcccacctcagaaccccttccacagttcccttaaagttcctttcctcatttacatcaggatcttcacaatggggacccctggtcacctcccaacccaacaaacgctccaaatgagccgccactgcagaaactcattatggcccaggcaggacaggcacatccaagtatctgaccaggctgttccatctgccaggcaggtcctgccctctctccacccacctgtctaacccctgcatcctcaagaccctacttagctatggccctgtgtgaaaggtccctccccatgcacccacagccatttgttctctctcatgtggccctaacaggctggggttcctggagactccatggggagccaggcatgaagatggcatatacccatgtgtcactccccagaacgtgagctgcctgccctggcaccatacacaaagggactgacagccccagaatcccaaggggtgcacctatgcatatgggaaaggcatgtttacgggtgagaatggtccatcgttgggcttcaggaggcatctgacctgacgcacgcctttgtcactttgtccttgtggcctgttgaaatgccactcctgctttacaaattcaccaactgttgcatgagtcatttccacctcaatgagtaccaggtccttgaggatggggaaaagtaagccaccactgtgggggtcctgggctcctaggtgcagaagaggctccagaaacaggccaggtcgtgggccatgaccccacactagccctctggtccctcacacgggtggattggggggctgtgtcacgggatcttaggatcttcaagacaaagacccaggacaagaacacaagcccactcccattcttcacaggcctcgagaaatctttgggcaatgaagtcagactgtgccaaagcccatgtttctgtctctccaaggcccctggcccccactgcctagcctaggtcaggtcatgtgggcaagcgagcccccacagcctcacagcccctaccccagggccagggcaaactcctgccctgtccccctccattcctgccctccctccttccacaaactgcaccagctggggagaaatccttcagccgacagaatgaggtgaaaatagtgcaattttaggctttgtaactgagattagggcaggtggccacccattctccccttcctcaggccagcctctgacacaatgaccctggaagcctggcagccctccgtaatggtcagcatcctcccctgccatccccaacccacaccatgagctcagccagggcaggggcagcctctgtctcattcaccacagaatccacagaacccagcacagagtatgagctcagtaaattctcctcatacatgactgcactgactggaccgggcacatgctacagggcaacacccacggctcagctggccctggctttggatctcagtcccacctcttcaagctgtccagcgtggggcacatcggctacagccttgccaaatgaaggcttgccaggatgaagaggtgaagacaggacaagcacagtatgtggcacacaggaggcctctgataacatcagtccccttccctaaagacctgggcagtccctgtcactggggcctcacatttcatgtcgagaattcactatttctcagcactgatttcaaataaagccaccaagagtctgacgaggcaacatggcagagttctgagggtggagtgaacaaaaggtcattttttacagaaaactcaggatctcccctctgcacagtgctaaagccctgtctcaaagttcagagcccggaaggtgcagagatgtggcccttggaaatcaagcccttaagaaaacagcccagctgtgtagggccggaagccccaggctgcagtcctgtggtctggaggcagccaatattcaggtgagagatgtgcccagctgccggtgggtccagggggcacggagcccccaccgtccctggcccaggtctaggactaagtcagtgggcccaggccagctccaagggccacagctcctcactcgggggccgcgccggagcagccgcagcagctggggcgccgcagggactgcatgacagcccgcagtggccccctccggccctccacagacaggctgtcctcgctggcgggcgcccgctgcagctgctcaaactgcatctccaggtgcttctggatggccacaccgagcacctccaggtccaccgcagctccgtacacctcccatgtcatgccctcagcatcccatcgcacatcccgcacaggggacggcacctcctccaggctggaccccagagttacctctgggaacacatgcagggctgcaggcgcttccagggacggactggtggccacagccttgcaggccgccactggggccgcctgcacaccagcatcctgggctgacagcggggatgcctctgcaggggccaagtcattggctgaggtcatggtccacacatctttggtcctagagccaggctctgggactaacccagcgggaccccaaaggtgggcacagcaatgggaatgcccagggagccccccagacaacctacagtggatcttcaccccatgctgagcctgcagcccagactcgctcactgacgccactagtttgggaaaggccaggatccctgtggcaggtagggcatggcagcagccaccagccctcacctccctcatgccacagagtagagcagctgggggcagagcatggcaggtggtggtagccagctgttcagcagctttgggctcagcctgggcactgctgctgtgggcagttgtgtcccccaggtctagtggtggcactgacaactgactcgcccccagcatccaggctgagttagaagtctcatcctcaggagccaggtccctttccaggcctgcaggggcctggccaccctggccagaagtaccacctggctgcagctgagccctgtggacagggctgctgccaagggctgagcagctgagactggccttccgagcaccactgtgtccccgcatctgggtgctacggaccaggtctgaatggctcctctgcatagcagcagcactaggggcccgcaggcgacacaggtcactgccgcccatggtggacacattgcccacagtgctgctccaccagtggcctccagcactgggtcgcgccttggggccagaggcccgtgctggcttcatgctctcaggcgggttcccctcttcctccggggcctggggtctggtgctggcctcgcccagctgggcctgccacacggtgctgctggcagtcttgcggagctctggcctctgttcccggccttcacccagcaggctggaagagctctgggacaggggctgaaggcgggggctcaggggtgcccagggacccggctcggggcggctggagctcatggctgcctctagctccaggggcaaggagaggccccatgcatcagctttttccatgagggactcattcagcatctggtcattgattccacagcatctcctgagcccctactgcgtgcccagctgtagggctagggaacatgggattcattcagacctttctgtacccctgatgtgtcgtcggcactcagaggattatctgctgtgtgcctgaccaagagaacaagcaaatacaagaacacacccacagaggagggcactgagtgccaaaaatggggtctgagggagggcaccaccaaggcaggagagctcacggagggtgagagatgagaaaaggcttcctggaggaccagccacgtaagtcaggcctggagtgagagaagcaagaaggtgttcaggtggagagcggagtgggcaggaggaaagaggccatgtgtccagagcatatgaggggagcagtggggtcaaagtgtctgggccacctcggccctggccacagcagtgaattagggagatcactctgggactccttgccaggcaggagaggtgggagaaacagggtggggacaggaggcagcagctgcatttgggcaatcccagccctgccctcccagcctaggctgataaagacttccaggcaacaacctccccgaccaggtgagcaaggctacccgagaggaaattcgggaagggctgtgggactcggtttctgtgtaattacaaatgtcctggcagcccagcactcaggagatggctggtggctgctgagccacagtgaggatgatactggtgctgtagtccctgagactccagctctgcacaacttcctgcgatgatggaaagattctaccctgtgctgtccaataggtaggcaccaatggcatgtgggtaccaagcactcagcagggggctactgcaactgagacactgaatgtttaagttttatttgaatctaactggccacatgaggctaatggctaccgtacaggactgtgcagctctgaacacagccccggcctggtaaggatgtcccatcccagctgcttcacggggctgaagccagacttgtccctgggaggatcaggaagaggaggagtagccaagagagaaatctgacccagaccctgccctcaatgagctctaagatggacatacaaacaaaggagggcaataaagcccgtaacagcgatgataataacagctgccagggcctgatcactcgccaagggccagacacgtgccacatcctttgcatacattgtctcatataactgtgcaagcaacctcttgagacagtcattatctccattctacagacaggagaattccataagctcagagaggctcagtgacccccaagggcacacacctgtggggcagctgagctcctctccccttcgagcactgagcaggcctatgcctcgcagctctcaccctttttactgatctggcctggccctgccaatcgtgctcatgacatgccatggaacaagtcactgagtggatctccacctgcccaacatgcttcttagcagctcctgaggctgcaagaatgaggagggcaggaggtgttcctcctgactgggacagctgtggtcactgccagcccctggcagggagacaaccactcagttgcaggtccaagaccccagggaggccccatctggacatccacacagcctctggccaaaccccaccaccctcccagggaggggggccataaacagccaggccagcagcctctggcccctgaggagacaggtggaatgaggtcctcagacccccaccaagacccactgagaagccatgagcaatgagcatcccactgtgcctgtctcaccagagggctgcccagcacccagggctagtcatcacccagagacccccgtgtgggctatgtatctattggttcccttccccattccccctccacaagtggcaggtgacaaaactgaggcctggagcagctcagaaatgtcaaagaacacacagctgaaagtggctaattcagaaccccaatggattggcctggctaactacaacctggccttcccagctcagaaggaaggaagggctctgaggggagtactgggggaaagaggcttccacactgcctgtcacagtgctgtggactgggccagaggaggggcctcccagggagccaggggtgaggaggaaggggcagggctctgcttccaatgggggctcttccccttcctgtgcatgtactcacaggtggacccctaacttctttgagcctcagtttcttcaatcttaatgttctctctcctgccccatttgatgccgaagttgctatggttgtggccgatgtcccgtggccaatgccaggctgtcctgctgcctcaggttccacctgtcagcaactggaagatcaaccaccctctcgcccgccggggccgcgcaggcgggggaagcgctgctcctgcggccgccacaggtgccaggtgccgcggcccaagatggagccagagccgacctggcctgggcgcgagacgccgcccgccgccgtcggcccggcc

SEQ ID NO: 15480 - RNA, 9212 nt, Homo sapiens
  source 1..9212: mol_type = other RNA
gctgggattacaggcatgagccactgtaccaggctgagtccacacttctaagcttgctgttgctctcagacttgcagaacaacctattaaacagaagtaggtaaaagttgagaaagggaagtggccaccacagaaccagttctgctgagaacgaggactcgagtcaggctatgctaccctccttccatggccatgggaaaaaggggtgtgtgctgttggtgtgagagatctggatcttaacagatcagacttaaactaatttgcccatgatgaccgtgtggatttggagggacctgggaatctcacagacctatgggatgtcccagtgatatgtcctgggcttcataccagccctgccctgcctgacaagttggatgaaaactgataaaggacttgtcatagcttcagatggcaaaaccaggccaggccagaatgaaaaaggagaaggaatttaacatgggcaaatgccaagctctgcatttaactaaccaaggctgcttggcgtgaacaaaactgagacagagcaatgcatggagaaaagggttgggcatttgtgggctacaagcttggcatgacatggatgcaaatgtcaatgggtgcacccccagatgcctgtgactccctctggtggtttctgtgcacaacttcccccaaaataggccctacgactccagcagaaacctaccctggggctcctagagcttcctagcctgcctgccagagagcagaagtgcctggaggctacatcttcacccctgggtagtccttactctgaggtgggactgcatccagggctcccctttagggtctgacttggactgaaatcacaccctgccttgccttctgcccctcccttaacttgctctcccctccctaataactccagcatcctcatctcagcagaagcttctggggaacccagcccaagatgagtggtgagggctagggtagccctcctcaatgcactctgggaactacattttcagaagccccagccagagggccaagtcccaggcagggtgcaaagctgtggggcgaggaacctggaaagaggctctgaacaagggacttttaaggaagtgggatgtgggctgtgatcacagccaagctggcagggtaagaggtggcccctgaatgtggctatgagaggggtgcccaacactaccagcctgtgtgctgagcactaactcagtgccaggcactacttgggttattctatttaatctccacaccaagcatgtgaaggaggcaccattgtcatccccatcttacagatgaggaagatgatcaaggcttgtaacttgcccaagatcacatggctataggtgtggatcctatatatccagattcaaactccagctttagcccactaagctacggtggccaaccccagcccaaagtgttgggacctgcgtgtagaagaccccttcagcccttgtaaagttaggatctagcatgtctaaggggacagagacccaatccaggtgacacaggaggtaagatcacagtggaacaggccatccctgcttttccaccaccaccagcactgtgacctcagaccagctctactctatgagtttcttgtgacagtgatggcagcctggggccagacaagggatgcgtgtcttgtgtcctggacacaagacaggcaggcccagaggggacaagctatatgaagagaggcttcagctgtcgggggtcctgaatgccatggaaggagagcaggtgggcagaagcagggagcccctggagcagacagaggggggattcctgctgaggcaaggggctctaggactccagggtttatgctccaaagaacagaatttaccaggacaaaataaacaagaccagtcaggaccgatgccccatccctgctggggtctggcaaagctctcacctccaaatttgtatctgttttgaattcaaagccaaacaaacacatcaacagtgaactccaacacctcccagagcagggcctgaaagggacccagaaagtctggccagaaatctagagtccaaggggaggagatctgtaaactaaaccgctggccatgctctggggccctaaaccactgcaggcatcagggctgttccaggagagggcacagcaaagggggttgggaggggtctccagttccaatcagaaatgaggctgcagtcacttcaggtagacctgtcagcagcagctgtgcaactgggctagggagacaaggatcgtggtttagccaggagaatcatctggggccccagccaagacacaggtgttggatttcagcaccgctctgcaaatactcatctcagtgacgatgaggtgagtgggagcttggctgagcccagcccggcctgccatcctggcaagccagggcagcatggaggtagcacagagtggcacccagccagcgtgaatgcataagaatctgcacgtgacacagaagaaagtctcttcatgaagtaggtttcactggtcccagccaaaccctgtggcaggtggccctttctgcacctgctgaacatgccattcaccttgacccaggtagtggcctcaccctcctcttgctcaaactggaaacctcagcatcctgaaatgcctcctccccaaatccattgcacacatgtgtgcctgtgtatgcgtgtgtgtgcacgtgtatgaacccagcccccagctgcccactccattgcccctaaacaggcccctccttggtgtcacctggcacatctccactggaagccaaatggatatttctaaactgaaatctggtcccacctcagaaccccttccacagttcccttaaagttcctttcctcatttacatcaggatcttcacaatggggacccctggtcacctcccaacccaacaaacgctccaaatgagccgccactgcagaaactcattatggcccaggcaggacaggcacatccaagtatctgaccaggctgttccatctgccaggcaggtcctgccctctctccacccacctgtctaacccctgcatcctcaagaccctacttagctatggccctgtgtgaaaggtccctccccatgcacccacagccatttgttctctctcatgtggccctaacaggctggggttcctggagactccatggggagccaggcatgaagatggcatatacccatgtgtcactccccagaacgtgagctgcctgccctggcaccatacacaaagggactgacagccccagaatcccaaggggtgcacctatgcatatgggaaaggcatgtttacgggtgagaatggtccatcgttgggcttcaggaggcatctgacctgacgcacgcctttgtcactttgtccttgtggcctgttgaaatgccactcctgctttacaaattcaccaactgttgcatgagtcatttccacctcaatgagtaccaggtccttgaggatggggaaaagtaagccaccactgtgggggtcctgggctcctaggtgcagaagaggctccagaaacaggccaggtcgtgggccatgaccccacactagccctctggtccctcacacgggtggattggggggctgtgtcacgggatcttaggatcttcaagacaaagacccaggacaagaacacaagcccactcccattcttcacaggcctcgagaaatctttgggcaatgaagtcagactgtgccaaagcccatgtttctgtctctccaaggcccctggcccccactgcctagcctaggtcaggtcatgtgggcaagcgagcccccacagcctcacagcccctaccccagggccagggcaaactcctgccctgtccccctccattcctgccctccctccttccacaaactgcaccagctggggagaaatccttcagccgacagaatgaggtgaaaatagtgcaattttaggctttgtaactgagattagggcaggtggccacccattctccccttcctcaggccagcctctgacacaatgaccctggaagcctggcagccctccgtaatggtcagcatcctcccctgccatccccaacccacaccatgagctcagccagggcaggggcagcctctgtctcattcaccacagaatccacagaacccagcacagagtatgagctcagtaaattctcctcatacatgactgcactgactggaccgggcacatgctacagggcaacacccacggctcagctggccctggctttggatctcagtcccacctcttcaagctgtccagcgtggggcacatcggctacagccttgccaaatgaaggcttgccaggatgaagaggtgaagacaggacaagcacagtatgtggcacacaggaggcctctgataacatcagtccccttccctaaagacctgggcagtccctgtcactggggcctcacatttcatgtcgagaattcactatttctcagcactgatttcaaataaagccaccaagagtctgacgaggcaacatggcagagttctgagggtggagtgaacaaaaggtcattttttacagaaaactcaggatctcccctctgcacagtgctaaagccctgtctcaaagttcagagcccggaaggtgcagagatgtggcccttggaaatcaagcccttaagaaaacagcccagctgtgtagggccggaagccccaggctgcagtcctgtggtctggaggcagccaatattcaggtgagagatgtgcccagctgccggtgggtccagggggcacggagcccccaccgtccctggcccaggtctaggactaagtcagtgggcccaggccagctccaagggccacagctcctcactcgggggccgcgccggagcagccgcagcagctggggcgccgcagggactgcatgacagcccgcagtggccccctccggccctccacagacaggctgtcctcgctggcgggcgcccgctgcagctgctcaaactgcatctccaggtgcttctggatggccacaccgagcacctccaggtccaccgcagctccgtacacctcccatgtcatgccctcagcatcccatcgcacatcccgcacaggggacggcacctcctccaggctggaccccagagttacctctgggaacacatgcagggctgcaggcgcttccagggacggactggtggccacagccttgcaggccgccactggggccgcctgcacaccagcatcctgggctgacagcggggatgcctctgcaggggccaagtcattggctgaggtcatggtccacacatctttggtcctagagccaggctctgggactaacccagcgggaccccaaaggtgggcacagcaatgggaatgcccagggagccccccagacaacctacagtggatcttcaccccatgctgagcctgcagcccagactcgctcactgacgccactagtttgggaaaggccaggatccctgtggcaggtagggcatggcagcagccaccagccctcacctccctcatgccacagagtagagcagctgggggcagagcatggcaggtggtggtagccagctgttcagcagctttgggctcagcctgggcactgctgctgtgggcagttgtgtcccccaggtctagtggtggcactgacaactgactcgcccccagcatccaggctgagttagaagtctcatcctcaggagccaggtccctttccaggcctgcaggggcctggccaccctggccagaagtaccacctggctgcagctgagccctgtggacagggctgctgccaagggctgagcagctgagactggccttccgagcaccactgtgtccccgcatctgggtgctacggaccaggtctgaatggctcctctgcatagcagcagcactaggggcccgcaggcgacacaggtcactgccgcccatggtggacacattgcccacagtgctgctccaccagtggcctccagcactgggtcgcgccttggggccagaggcccgtgctggcttcatgctctcaggcgggttcccctcttcctccggggcctggggtctggtgctggcctcgcccagctgggcctgccacacggtgctgctggcagtcttgcggagctctggcctctgttcccggccttcacccagcaggctggaagagctctgggacaggggctgaaggcgggggctcaggggtgcccagggacccggctcggggcggctggagctcatggctgcctctagctccaggggcaaggagaggccccatgcatcagctttttccatgagggactcattcagcatctggtcattgattccacagcatctcctgagcccctactgcgtgcccagctgtagggctagggaacatgggattcattcagacctttctgtacccctgatgtgtcgtcggcactcagaggattatctgctgtgtgcctgaccaagagaacaagcaaatacaagaacacacccacagaggagggcactgagtgccaaaaatggggtctgagggagggcaccaccaaggcaggagagctcacggagggtgagagatgagaaaaggcttcctggaggaccagccacgtaagtcaggcctggagtgagagaagcaagaaggtgttcaggtggagagcggagtgggcaggaggaaagaggccatgtgtccagagcatatgaggggagcagtggggtcaaagtgtctgggccacctcggccctggccacagcagtgaattagggagatcactctgggactccttgccaggcaggagaggtgggagaaacagggtggggacaggaggcagcagctgcatttgggcaatcccagccctgccctcccagcctaggctgataaagacttccaggcaacaacctccccgaccaggtgagcaaggctacccgagaggaaattcgggaagggctgtgggactcggtttctgtgtaattacaaatgtcctggcagcccagcactcaggagatggctggtggctgctgagccacagtgaggatgatactggtgctgtagtccctgagactccagctctgcacaacttcctgcgatgatggaaagattctaccctgtgctgtccaataggtaggcaccaatggcatgtgggtaccaagcactcagcagggggctactgcaactgagacactgaatgtttaagttttatttgaatctaactggccacatgaggctaatggctaccgtacaggactgtgcagctctgaacacagccccggcctggtaaggatgtcccatcccagctgcttcacggggctgaagccagacttgtccctgggaggatcaggaagaggaggagtagccaagagagaaatctgacccagaccctgccctcaatgagctctaagatggacatacaaacaaaggagggcaataaagcccgtaacagcgatgataataacagctgccagggcctgatcactcgccaagggccagacacgtgccacatcctttgcatacattgtctcatataactgtgcaagcaacctcttgagacagtcattatctccattctacagacaggagaattccataagctcagagaggctcagtgacccccaagggcacacacctgtggggcagctgagctcctctccccttcgagcactgagcaggcctatgcctcgcagctctcaccctttttactgatctggcctggccctgccaatcgtgctcatgacatgccatggaacaagtcactgagtggatctccacctgcccaacatgcttcttagcagctcctgaggctgcaagaatgaggagggcaggaggtgttcctcctgactgggacagctgtggtcactgccagcccctggcagggagacaaccactcagttgcaggtccaagaccccagggaggccccatctggacatccacacagcctctggccaaaccccaccaccctcccagggaggggggccataaacagccaggccagcagcctctggcccctgaggagacaggtggaatgaggtcctcagacccccaccaagacccactgagaagccatgagcaatgagcatcccactgtgcctgtctcaccagagggctgcccagcacccagggctagtcatcacccagagacccccgtgtgggctatgtatctattggttcccttccccattccccctccacaagtggcaggtgacaaaactgaggcctggagcagctcagaaatgtcaaagaacacacagctgaaagtggctaattcagaaccccaatggattggcctggctaactacaacctggccttcccagctcagaaggaaggaagggctctgaggggagtactgggggaaagaggcttccacactgcctgtcacagtgctgtggactgggccagaggaggggcctcccagggagccaggggtgaggaggaaggggcagggctctgcttccaatgggggctcttccccttcctgtgcatgtactcacaggtggacccctaacttctttgagcctcagtttcttcaatcttaatgttctctctcctgccccatttgatgccgaagttgctatggttgtggccgatgtcccgtggccaatgccaggctgtcctgctgcctcaggttccacctgtcagcaactggaagatcaaccacctctcaaggaccaggcaggaatgcacacagcacaaacccccattgcacagtggggatacagcaccctccaggaggtggtttaatccaccccagagtgaacggggcctgataggaacactcagggccaactctgggcaaagcagcaggcagcattcctaaagggagggtttggaggagacaaaacctgcccttcacaatgaacgtgccttaagggctacatgccccgggtcacaagctgtgccaggaaagggttctggggtaactgtggggtcagtggccccatggatgaggctctgctcaccaggaagaggcctaggcgcccaacagcccctgagcttcctcccctggggaggatttgcccacaatccctggggggcacctaggtggagagggtgccccggcctagaagcagcctaggcggccggtgtgtccctatctgcacgctcacaagcactcatgccccagcctgggacacacaggcccgtatgcagtaacagcgtctacccagctgcactctgcacgccaagcacaggccgcccctgctgcggggccaaaggcctgaaagcaccgcaccacgcagcctcgcccagaatagctcccctcccgcccctcctgcacaaagcccacccggacttagggagaagggggctcaatacgggcccgaaac

SEQ ID NO: 15481 - RNA, 8960 nt, Homo sapiens
  source 1..8960: mol_type = other RNA
gctgggattacaggcatgagccactgtaccaggctgagtccacacttctaagcttgctgttgctctcagacttgcagaacaacctattaaacagaagtaggtaaaagttgagaaagggaagtggccaccacagaaccagttctgctgagaacgaggactcgagtcaggctatgctaccctccttccatggccatgggaaaaaggggtgtgtgctgttggtgtgagagatctggatcttaacagatcagacttaaactaatttgcccatgatgaccgtgtggatttggagggacctgggaatctcacagacctatgggatgtcccagtgatatgtcctgggcttcataccagccctgccctgcctgacaagttggatgaaaactgataaaggacttgtcatagcttcagatggcaaaaccaggccaggccagaatgaaaaaggagaaggaatttaacatgggcaaatgccaagctctgcatttaactaaccaaggctgcttggcgtgaacaaaactgagacagagcaatgcatggagaaaagggttgggcatttgtgggctacaagcttggcatgacatggatgcaaatgtcaatgggtgcacccccagatgcctgtgactccctctggtggtttctgtgcacaacttcccccaaaataggccctacgactccagcagaaacctaccctggggctcctagagcttcctagcctgcctgccagagagcagaagtgcctggaggctacatcttcacccctgggtagtccttactctgaggtgggactgcatccagggctcccctttagggtctgacttggactgaaatcacaccctgccttgccttctgcccctcccttaacttgctctcccctccctaataactccagcatcctcatctcagcagaagcttctggggaacccagcccaagatgagtggtgagggctagggtagccctcctcaatgcactctgggaactacattttcagaagccccagccagagggccaagtcccaggcagggtgcaaagctgtggggcgaggaacctggaaagaggctctgaacaagggacttttaaggaagtgggatgtgggctgtgatcacagccaagctggcagggtaagaggtggcccctgaatgtggctatgagaggggtgcccaacactaccagcctgtgtgctgagcactaactcagtgccaggcactacttgggttattctatttaatctccacaccaagcatgtgaaggaggcaccattgtcatccccatcttacagatgaggaagatgatcaaggcttgtaacttgcccaagatcacatggctataggtgtggatcctatatatccagattcaaactccagctttagcccactaagctacggtggccaaccccagcccaaagtgttgggacctgcgtgtagaagaccccttcagcccttgtaaagttaggatctagcatgtctaaggggacagagacccaatccaggtgacacaggaggtaagatcacagtggaacaggccatccctgcttttccaccaccaccagcactgtgacctcagaccagctctactctatgagtttcttgtgacagtgatggcagcctggggccagacaagggatgcgtgtcttgtgtcctggacacaagacaggcaggcccagaggggacaagctatatgaagagaggcttcagctgtcgggggtcctgaatgccatggaaggagagcaggtgggcagaagcagggagcccctggagcagacagaggggggattcctgctgaggcaaggggctctaggactccagggtttatgctccaaagaacagaatttaccaggacaaaataaacaagaccagtcaggaccgatgccccatccctgctggggtctggcaaagctctcacctccaaatttgtatctgttttgaattcaaagccaaacaaacacatcaacagtgaactccaacacctcccagagcagggcctgaaagggacccagaaagtctggccagaaatctagagtccaaggggaggagatctgtaaactaaaccgctggccatgctctggggccctaaaccactgcaggcatcagggctgttccaggagagggcacagcaaagggggttgggaggggtctccagttccaatcagaaatgaggctgcagtcacttcaggtagacctgtcagcagcagctgtgcaactgggctagggagacaaggatcgtggtttagccaggagaatcatctggggccccagccaagacacaggtgttggatttcagcaccgctctgcaaatactcatctcagtgacgatgaggtgagtgggagcttggctgagcccagcccggcctgccatcctggcaagccagggcagcatggaggtagcacagagtggcacccagccagcgtgaatgcataagaatctgcacgtgacacagaagaaagtctcttcatgaagtaggtttcactggtcccagccaaaccctgtggcaggtggccctttctgcacctgctgaacatgccattcaccttgacccaggtagtggcctcaccctcctcttgctcaaactggaaacctcagcatcctgaaatgcctcctccccaaatccattgcacacatgtgtgcctgtgtatgcgtgtgtgtgcacgtgtatgaacccagcccccagctgcccactccattgcccctaaacaggcccctccttggtgtcacctggcacatctccactggaagccaaatggatatttctaaactgaaatctggtcccacctcagaaccccttccacagttcccttaaagttcctttcctcatttacatcaggatcttcacaatggggacccctggtcacctcccaacccaacaaacgctccaaatgagccgccactgcagaaactcattatggcccaggcaggacaggcacatccaagtatctgaccaggctgttccatctgccaggcaggtcctgccctctctccacccacctgtctaacccctgcatcctcaagaccctacttagctatggccctgtgtgaaaggtccctccccatgcacccacagccatttgttctctctcatgtggccctaacaggctggggttcctggagactccatggggagccaggcatgaagatggcatatacccatgtgtcactccccagaacgtgagctgcctgccctggcaccatacacaaagggactgacagccccagaatcccaaggggtgcacctatgcatatgggaaaggcatgtttacgggtgagaatggtccatcgttgggcttcaggaggcatctgacctgacgcacgcctttgtcactttgtccttgtggcctgttgaaatgccactcctgctttacaaattcaccaactgttgcatgagtcatttccacctcaatgagtaccaggtccttgaggatggggaaaagtaagccaccactgtgggggtcctgggctcctaggtgcagaagaggctccagaaacaggccaggtcgtgggccatgaccccacactagccctctggtccctcacacgggtggattggggggctgtgtcacgggatcttaggatcttcaagacaaagacccaggacaagaacacaagcccactcccattcttcacaggcctcgagaaatctttgggcaatgaagtcagactgtgccaaagcccatgtttctgtctctccaaggcccctggcccccactgcctagcctaggtcaggtcatgtgggcaagcgagcccccacagcctcacagcccctaccccagggccagggcaaactcctgccctgtccccctccattcctgccctccctccttccacaaactgcaccagctggggagaaatccttcagccgacagaatgaggtgaaaatagtgcaattttaggctttgtaactgagattagggcaggtggccacccattctccccttcctcaggccagcctctgacacaatgaccctggaagcctggcagccctccgtaatggtcagcatcctcccctgccatccccaacccacaccatgagctcagccagggcaggggcagcctctgtctcattcaccacagaatccacagaacccagcacagagtatgagctcagtaaattctcctcatacatgactgcactgactggaccgggcacatgctacagggcaacacccacggctcagctggccctggctttggatctcagtcccacctcttcaagctgtccagcgtggggcacatcggctacagccttgccaaatgaaggcttgccaggatgaagaggtgaagacaggacaagcacagtatgtggcacacaggaggcctctgataacatcagtccccttccctaaagacctgggcagtccctgtcactggggcctcacatttcatgtcgagaattcactatttctcagcactgatttcaaataaagccaccaagagtctgacgaggcaacatggcagagttctgagggtggagtgaacaaaaggtcattttttacagaaaactcaggatctcccctctgcacagtgctaaagccctgtctcaaagttcagagcccggaaggtgcagagatgtggcccttggaaatcaagcccttaagaaaacagcccagctgtgtagggccggaagccccaggctgcagtcctgtggtctggaggcagccaatattcaggtgagagatgtgcccagctgccggtgggtccagggggcacggagcccccaccgtccctggcccaggtctaggactaagtcagtgggcccaggccagctccaagggccacagctcctcactcgggggccgcgccggagcagccgcagcagctggggcgccgcagggactgcatgacagcccgcagtggccccctccggccctccacagacaggctgtcctcgctggcgggcgcccgctgcagctgctcaaactgcatctccaggtgcttctggatggccacaccgagcacctccaggtccaccgcagctccgtacacctcccatgtcatgccctcagcatcccatcgcacatcccgcacaggggacggcacctcctccaggctggaccccagagttacctctgggaacacatgcagggctgcaggcgcttccagggacggactggtggccacagccttgcaggccgccactggggccgcctgcacaccagcatcctgggctgacagcggggatgcctctgcaggggccaagtcattggctgaggtcatggtccacacatctttggtcctagagccaggctctgggactaacccagcgggaccccaaaggtgggcacagcaatgggaatgcccagggagccccccagacaacctacagtggatcttcaccccatgctgagcctgcagcccagactcgctcactgacgccactagtttgggaaaggccaggatccctgtggcaggtagggcatggcagcagccaccagccctcacctccctcatgccacagagtagagcagctgggggcagagcatggcaggtggtggtagccagctgttcagcagctttgggctcagcctgggcactgctgctgtgggcagttgtgtcccccaggtctagtggtggcactgacaactgactcgcccccagcatccaggctgagttagaagtctcatcctcaggagccaggtccctttccaggcctgcaggggcctggccaccctggccagaagtaccacctggctgcagctgagccctgtggacagggctgctgccaagggctgagcagctgagactggccttccgagcaccactgtgtccccgcatctgggtgctacggaccaggtctgaatggctcctctgcatagcagcagcactaggggcccgcaggcgacacaggtcactgccgcccatggtggacacattgcccacagtgctgctccaccagtggcctccagcactgggtcgcgccttggggccagaggcccgtgctggcttcatgctctcaggcgggttcccctcttcctccggggcctggggtctggtgctggcctcgcccagctgggcctgccacacggtgctgctggcagtcttgcggagctctggcctctgttcccggccttcacccagcaggctggaagagctctgggacaggggctgaaggcgggggctcaggggtgcccagggacccggctcggggcggctggagctcatggctgcctctagctccaggggcaaggagaggccccatgcatcagctttttccatgagggactcattcagcatctggtcattgattccacagcatctcctgagcccctactgcgtgcccagctgtagggctagggaacatgggattcattcagacctttctgtacccctgatgtgtcgtcggcactcagaggattatctgctgtgtgcctgaccaagagaacaagcaaatacaagaacacacccacagaggagggcactgagtgccaaaaatggggtctgagggagggcaccaccaaggcaggagagctcacggagggtgagagatgagaaaaggcttcctggaggaccagccacgtaagtcaggcctggagtgagagaagcaagaaggtgttcaggtggagagcggagtgggcaggaggaaagaggccatgtgtccagagcatatgaggggagcagtggggtcaaagtgtctgggccacctcggccctggccacagcagtgaattagggagatcactctgggactccttgccaggcaggagaggtgggagaaacagggtggggacaggaggcagcagctgcatttgggcaatcccagccctgccctcccagcctaggctgataaagacttccaggcaacaacctccccgaccaggtgagcaaggctacccgagaggaaattcgggaagggctgtgggactcggtttctgtgtaattacaaatgtcctggcagcccagcactcaggagatggctggtggctgctgagccacagtgaggatgatactggtgctgtagtccctgagactccagctctgcacaacttcctgcgatgatggaaagattctaccctgtgctgtccaataggtaggcaccaatggcatgtgggtaccaagcactcagcagggggctactgcaactgagacactgaatgtttaagttttatttgaatctaactggccacatgaggctaatggctaccgtacaggactgtgcagctctgaacacagccccggcctggtaaggatgtcccatcccagctgcttcacggggctgaagccagacttgtccctgggaggatcaggaagaggaggagtagccaagagagaaatctgacccagaccctgccctcaatgagctctaagatggacatacaaacaaaggagggcaataaagcccgtaacagcgatgataataacagctgccagggcctgatcactcgccaagggccagacacgtgccacatcctttgcatacattgtctcatataactgtgcaagcaacctcttgagacagtcattatctccattctacagacaggagaattccataagctcagagaggctcagtgacccccaagggcacacacctgtggggcagctgagctcctctccccttcgagcactgagcaggcctatgcctcgcagctctcaccctttttactgatctggcctggccctgccaatcgtgctcatgacatgccatggaacaagtcactgagtggatctccacctgcccaacatgcttcttagcagctcctgaggctgcaagaatgaggagggcaggaggtgttcctcctgactgggacagctgtggtcactgccagcccctggcagggagacaaccactcagttgcaggtccaagaccccagggaggccccatctggacatccacacagcctctggccaaaccccaccaccctcccagggaggggggccataaacagccaggccagcagcctctggcccctgaggagacaggtggaatgaggtcctcagacccccaccaagacccactgagaagccatgagcaatgagcatcccactgtgcctgtctcaccagagggctgcccagcacccagggctagtcatcacccagagacccccgtgtgggctatgtatctattggttcccttccccattccccctccacaagtggcaggtgacaaaactgaggcctggagcagctcagaaatgtcaaagaacacacagctgaaagtggctaattcagaaccccaatggattggcctggctaactacaacctggccttcccagctcagaaggaaggaagggctctgaggggagtactgggggaaagaggcttccacactgcctgtcacagtgctgtggactgggccagaggaggggcctcccagggagccaggggtgaggaggaaggggcagggctctgcttccaatgggggctcttccccttcctgtgcatgtactcacaggtggacccctaacttctttgagcctcagtttcttcaatcttaatgttctctctcctgccccatttgatgccgaagttgctatggttgtggccgatgtcccgtggccaatgccaggctgtcctgctgcctcaggttccacctgtcagcaactggaagatcaaccaccttctcaggagcaaaggcagcgactgcaggcaaatggggctgtgggccggggtaatgatgcgggacaggagaagccaaagggcagcaaggctgggggcggggtaggcggcgcagtaggctgagggaggggaaaaggaagaaggggagagggaggagcgatggcagcaggggtggaggccgaaggagacagggtcccggacagacttgtgaaaatgggaggatgggcagaggagacgtagaagaggggacaggacaggacaatgagaggcggagcgcggggagtgcgatgcggccaccgggggctctgggcgctgggcaggggccaggatgccgggggtctgagcgcaggcagcgggaaggagtgggttctgaggctcagcaagggggaggtgccgcccaccacgccccccgcccc

SEQ ID NO: 15482 - RNA, 8944 nt, Homo sapiens
  source 1..8944: mol_type = other RNA
gctgggattacaggcatgagccactgtaccaggctgagtccacacttctaagcttgctgttgctctcagacttgcagaacaacctattaaacagaagtaggtaaaagttgagaaagggaagtggccaccacagaaccagttctgctgagaacgaggactcgagtcaggctatgctaccctccttccatggccatgggaaaaaggggtgtgtgctgttggtgtgagagatctggatcttaacagatcagacttaaactaatttgcccatgatgaccgtgtggatttggagggacctgggaatctcacagacctatgggatgtcccagtgatatgtcctgggcttcataccagccctgccctgcctgacaagttggatgaaaactgataaaggacttgtcatagcttcagatggcaaaaccaggccaggccagaatgaaaaaggagaaggaatttaacatgggcaaatgccaagctctgcatttaactaaccaaggctgcttggcgtgaacaaaactgagacagagcaatgcatggagaaaagggttgggcatttgtgggctacaagcttggcatgacatggatgcaaatgtcaatgggtgcacccccagatgcctgtgactccctctggtggtttctgtgcacaacttcccccaaaataggccctacgactccagcagaaacctaccctggggctcctagagcttcctagcctgcctgccagagagcagaagtgcctggaggctacatcttcacccctgggtagtccttactctgaggtgggactgcatccagggctcccctttagggtctgacttggactgaaatcacaccctgccttgccttctgcccctcccttaacttgctctcccctccctaataactccagcatcctcatctcagcagaagcttctggggaacccagcccaagatgagtggtgagggctagggtagccctcctcaatgcactctgggaactacattttcagaagccccagccagagggccaagtcccaggcagggtgcaaagctgtggggcgaggaacctggaaagaggctctgaacaagggacttttaaggaagtgggatgtgggctgtgatcacagccaagctggcagggtaagaggtggcccctgaatgtggctatgagaggggtgcccaacactaccagcctgtgtgctgagcactaactcagtgccaggcactacttgggttattctatttaatctccacaccaagcatgtgaaggaggcaccattgtcatccccatcttacagatgaggaagatgatcaaggcttgtaacttgcccaagatcacatggctataggtgtggatcctatatatccagattcaaactccagctttagcccactaagctacggtggccaaccccagcccaaagtgttgggacctgcgtgtagaagaccccttcagcccttgtaaagttaggatctagcatgtctaaggggacagagacccaatccaggtgacacaggaggtaagatcacagtggaacaggccatccctgcttttccaccaccaccagcactgtgacctcagaccagctctactctatgagtttcttgtgacagtgatggcagcctggggccagacaagggatgcgtgtcttgtgtcctggacacaagacaggcaggcccagaggggacaagctatatgaagagaggcttcagctgtcgggggtcctgaatgccatggaaggagagcaggtgggcagaagcagggagcccctggagcagacagaggggggattcctgctgaggcaaggggctctaggactccagggtttatgctccaaagaacagaatttaccaggacaaaataaacaagaccagtcaggaccgatgccccatccctgctggggtctggcaaagctctcacctccaaatttgtatctgttttgaattcaaagccaaacaaacacatcaacagtgaactccaacacctcccagagcagggcctgaaagggacccagaaagtctggccagaaatctagagtccaaggggaggagatctgtaaactaaaccgctggccatgctctggggccctaaaccactgcaggcatcagggctgttccaggagagggcacagcaaagggggttgggaggggtctccagttccaatcagaaatgaggctgcagtcacttcaggtagacctgtcagcagcagctgtgcaactgggctagggagacaaggatcgtggtttagccaggagaatcatctggggccccagccaagacacaggtgttggatttcagcaccgctctgcaaatactcatctcagtgacgatgaggtgagtgggagcttggctgagcccagcccggcctgccatcctggcaagccagggcagcatggaggtagcacagagtggcacccagccagcgtgaatgcataagaatctgcacgtgacacagaagaaagtctcttcatgaagtaggtttcactggtcccagccaaaccctgtggcaggtggccctttctgcacctgctgaacatgccattcaccttgacccaggtagtggcctcaccctcctcttgctcaaactggaaacctcagcatcctgaaatgcctcctccccaaatccattgcacacatgtgtgcctgtgtatgcgtgtgtgtgcacgtgtatgaacccagcccccagctgcccactccattgcccctaaacaggcccctccttggtgtcacctggcacatctccactggaagccaaatggatatttctaaactgaaatctggtcccacctcagaaccccttccacagttcccttaaagttcctttcctcatttacatcaggatcttcacaatggggacccctggtcacctcccaacccaacaaacgctccaaatgagccgccactgcagaaactcattatggcccaggcaggacaggcacatccaagtatctgaccaggctgttccatctgccaggcaggtcctgccctctctccacccacctgtctaacccctgcatcctcaagaccctacttagctatggccctgtgtgaaaggtccctccccatgcacccacagccatttgttctctctcatgtggccctaacaggctggggttcctggagactccatggggagccaggcatgaagatggcatatacccatgtgtcactccccagaacgtgagctgcctgccctggcaccatacacaaagggactgacagccccagaatcccaaggggtgcacctatgcatatgggaaaggcatgtttacgggtgagaatggtccatcgttgggcttcaggaggcatctgacctgacgcacgcctttgtcactttgtccttgtggcctgttgaaatgccactcctgctttacaaattcaccaactgttgcatgagtcatttccacctcaatgagtaccaggtccttgaggatggggaaaagtaagccaccactgtgggggtcctgggctcctaggtgcagaagaggctccagaaacaggccaggtcgtgggccatgaccccacactagccctctggtccctcacacgggtggattggggggctgtgtcacgggatcttaggatcttcaagacaaagacccaggacaagaacacaagcccactcccattcttcacaggcctcgagaaatctttgggcaatgaagtcagactgtgccaaagcccatgtttctgtctctccaaggcccctggcccccactgcctagcctaggtcaggtcatgtgggcaagcgagcccccacagcctcacagcccctaccccagggccagggcaaactcctgccctgtccccctccattcctgccctccctccttccacaaactgcaccagctggggagaaatccttcagccgacagaatgaggtgaaaatagtgcaattttaggctttgtaactgagattagggcaggtggccacccattctccccttcctcaggccagcctctgacacaatgaccctggaagcctggcagccctccgtaatggtcagcatcctcccctgccatccccaacccacaccatgagctcagccagggcaggggcagcctctgtctcattcaccacagaatccacagaacccagcacagagtatgagctcagtaaattctcctcatacatgactgcactgactggaccgggcacatgctacagggcaacacccacggctcagctggccctggctttggatctcagtcccacctcttcaagctgtccagcgtggggcacatcggctacagccttgccaaatgaaggcttgccaggatgaagaggtgaagacaggacaagcacagtatgtggcacacaggaggcctctgataacatcagtccccttccctaaagacctgggcagtccctgtcactggggcctcacatttcatgtcgagaattcactatttctcagcactgatttcaaataaagccaccaagagtctgacgaggcaacatggcagagttctgagggtggagtgaacaaaaggtcattttttacagaaaactcaggatctcccctctgcacagtgctaaagccctgtctcaaagttcagagcccggaaggtgcagagatgtggcccttggaaatcaagcccttaagaaaacagcccagctgtgtagggccggaagccccaggctgcagtcctgtggtctggaggcagccaatattcaggtgagagatgtgcccagctgccggtgggtccagggggcacggagcccccaccgtccctggcccaggtctaggactaagtcagtgggcccaggccagctccaagggccacagctcctcactcgggggccgcgccggagcagccgcagcagctggggcgccgcagggactgcatgacagcccgcagtggccccctccggccctccacagacaggctgtcctcgctggcgggcgcccgctgcagctgctcaaactgcatctccaggtgcttctggatggccacaccgagcacctccaggtccaccgcagctccgtacacctcccatgtcatgccctcagcatcccatcgcacatcccgcacaggggacggcacctcctccaggctggaccccagagttacctctgggaacacatgcagggctgcaggcgcttccagggacggactggtggccacagccttgcaggccgccactggggccgcctgcacaccagcatcctgggctgacagcggggatgcctctgcaggggccaagtcattggctgaggtcatggtccacacatctttggtcctagagccaggctctgggactaacccagcgggaccccaaaggtgggcacagcaatgggaatgcccagggagccccccagacaacctacagtggatcttcaccccatgctgagcctgcagcccagactcgctcactgacgccactagtttgggaaaggccaggatccctgtggcaggtagggcatggcagcagccaccagccctcacctccctcatgccacagagtagagcagctgggggcagagcatggcaggtggtggtagccagctgttcagcagctttgggctcagcctgggcactgctgctgtgggcagttgtgtcccccaggtctagtggtggcactgacaactgactcgcccccagcatccaggctgagttagaagtctcatcctcaggagccaggtccctttccaggcctgcaggggcctggccaccctggccagaagtaccacctggctgcagctgagccctgtggacagggctgctgccaagggctgagcagctgagactggccttccgagcaccactgtgtccccgcatctgggtgctacggaccaggtctgaatggctcctctgcatagcagcagcactaggggcccgcaggcgacacaggtcactgccgcccatggtggacacattgcccacagtgctgctccaccagtggcctccagcactgggtcgcgccttggggccagaggcccgtgctggcttcatgctctcaggcgggttcccctcttcctccggggcctggggtctggtgctggcctcgcccagctgggcctgccacacggtgctgctggcagtcttgcggagctctggcctctgttcccggccttcacccagcaggctggaagagctctgggacaggggctgaaggcgggggctcaggggtgcccagggacccggctcggggcggctggagctcatggctgcctctagctccaggggcaaggagaggccccatgcatcagctttttccatgagggactcattcagcatctggtcattgattccacagcatctcctgagcccctactgcgtgcccagctgtagggctagggaacatgggattcattcagacctttctgtacccctgatgtgtcgtcggcactcagaggattatctgctgtgtgcctgaccaagagaacaagcaaatacaagaacacacccacagaggagggcactgagtgccaaaaatggggtctgagggagggcaccaccaaggcaggagagctcacggagggtgagagatgagaaaaggcttcctggaggaccagccacgtaagtcaggcctggagtgagagaagcaagaaggtgttcaggtggagagcggagtgggcaggaggaaagaggccatgtgtccagagcatatgaggggagcagtggggtcaaagtgtctgggccacctcggccctggccacagcagtgaattagggagatcactctgggactccttgccaggcaggagaggtgggagaaacagggtggggacaggaggcagcagctgcatttgggcaatcccagccctgccctcccagcctaggctgataaagacttccaggcaacaacctccccgaccaggtgagcaaggctacccgagaggaaattcgggaagggctgtgggactcggtttctgtgtaattacaaatgtcctggcagcccagcactcaggagatggctggtggctgctgagccacagtgaggatgatactggtgctgtagtccctgagactccagctctgcacaacttcctgcgatgatggaaagattctaccctgtgctgtccaataggtaggcaccaatggcatgtgggtaccaagcactcagcagggggctactgcaactgagacactgaatgtttaagttttatttgaatctaactggccacatgaggctaatggctaccgtacaggactgtgcagctctgaacacagccccggcctggtaaggatgtcccatcccagctgcttcacggggctgaagccagacttgtccctgggaggatcaggaagaggaggagtagccaagagagaaatctgacccagaccctgccctcaatgagctctaagatggacatacaaacaaaggagggcaataaagcccgtaacagcgatgataataacagctgccagggcctgatcactcgccaagggccagacacgtgccacatcctttgcatacattgtctcatataactgtgcaagcaacctcttgagacagtcattatctccattctacagacaggagaattccataagctcagagaggctcagtgacccccaagggcacacacctgtggggcagctgagctcctctccccttcgagcactgagcaggcctatgcctcgcagctctcaccctttttactgatctggcctggccctgccaatcgtgctcatgacatgccatggaacaagtcactgagtggatctccacctgcccaacatgcttcttagcagctcctgaggctgcaagaatgaggagggcaggaggtgttcctcctgactgggacagctgtggtcactgccagcccctggcagggagacaaccactcagttgcaggtccaagaccccagggaggccccatctggacatccacacagcctctggccaaaccccaccaccctcccagggaggggggccataaacagccaggccagcagcctctggcccctgaggagacaggtggaatgaggtcctcagacccccaccaagacccactgagaagccatgagcaatgagcatcccactgtgcctgtctcaccagagggctgcccagcacccagggctagtcatcacccagagacccccgtgtgggctatgtatctattggttcccttccccattccccctccacaagtggcaggtgacaaaactgaggcctggagcagctcagaaatgtcaaagaacacacagctgaaagtggctaattcagaaccccaatggattggcctggctaactacaacctggccttcccagctcagaaggaaggaagggctctgaggggagtactgggggaaagaggcttccacactgcctgtcacagtgctgtggactgggccagaggaggggcctcccagggagccaggggtgaggaggaaggggcagggctctgcttccaatgggggctcttccccttcctgtgcatgtactcacaggtggacccctaacttctttgagcctcagtttcttcaatcttaatgttctctctcctgccccatttgatgccgaagttgctatggttgtggccgatgtcccgtggccaatgccaggctgtcctgctgcctcaggttccacctgtcagcaacttctcaggagcaaaggcagcgactgcaggcaaatggggctgtgggccggggtaatgatgcgggacaggagaagccaaagggcagcaaggctgggggcggggtaggcggcgcagtaggctgagggaggggaaaaggaagaaggggagagggaggagcgatggcagcaggggtggaggccgaaggagacagggtcccggacagacttgtgaaaatgggaggatgggcagaggagacgtagaagaggggacaggacaggacaatgagaggcggagcgcggggagtgcgatgcggccaccgggggctctgggcgctgggcaggggccaggatgccgggggtctgagcgcaggcagcgggaaggagtgggttctgaggctcagcaagggggaggtgccgcccaccacgccccccgcccc

SEQ ID NO: 15483 - RNA, 6856 nt, Homo sapiens
  source 1..6856: mol_type = other RNA
gctgggattacaggcatgagccactgtaccaggctgagtccacacttctaagcttgctgttgctctcagacttgcagaacaacctattaaacagaagtaggtaaaagttgagaaagggaagtggccaccacagaaccagttctgctgagaacgaggactcgagtcaggctatgctaccctccttccatggccatgggaaaaaggggtgtgtgctgttggtgtgagagatctggatcttaacagatcagacttaaactaatttgcccatgatgaccgtgtggatttggagggacctgggaatctcacagacctatgggatgtcccagtgatatgtcctgggcttcataccagccctgccctgcctgacaagttggatgaaaactgataaaggacttgtcatagcttcagatggcaaaaccaggccaggccagaatgaaaaaggagaaggaatttaacatgggcaaatgccaagctctgcatttaactaaccaaggctgcttggcgtgaacaaaactgagacagagcaatgcatggagaaaagggttgggcatttgtgggctacaagcttggcatgacatggatgcaaatgtcaatgggtgcacccccagatgcctgtgactccctctggtggtttctgtgcacaacttcccccaaaataggccctacgactccagcagaaacctaccctggggctcctagagcttcctagcctgcctgccagagagcagaagtgcctggaggctacatcttcacccctgggtagtccttactctgaggtgggactgcatccagggctcccctttagggtctgacttggactgaaatcacaccctgccttgccttctgcccctcccttaacttgctctcccctccctaataactccagcatcctcatctcagcagaagcttctggggaacccagcccaagatgagtggtgagggctagggtagccctcctcaatgcactctgggaactacattttcagaagccccagccagagggccaagtcccaggcagggtgcaaagctgtggggcgaggaacctggaaagaggctctgaacaagggacttttaaggaagtgggatgtgggctgtgatcacagccaagctggcagggtaagaggtggcccctgaatgtggctatgagaggggtgcccaacactaccagcctgtgtgctgagcactaactcagtgccaggcactacttgggttattctatttaatctccacaccaagcatgtgaaggaggcaccattgtcatccccatcttacagatgaggaagatgatcaaggcttgtaacttgcccaagatcacatggctataggtgtggatcctatatatccagattcaaactccagctttagcccactaagctacggtggccaaccccagcccaaagtgttgggacctgcgtgtagaagaccccttcagcccttgtaaagttaggatctagcatgtctaaggggacagagacccaatccaggtgacacaggaggtaagatcacagtggaacaggccatccctgcttttccaccaccaccagcactgtgacctcagaccagctctactctatgagtttcttgtgacagtgatggcagcctggggccagacaagggatgcgtgtcttgtgtcctggacacaagacaggcaggcccagaggggacaagctatatgaagagaggcttcagctgtcgggggtcctgaatgccatggaaggagagcaggtgggcagaagcagggagcccctggagcagacagaggggggattcctgctgaggcaaggggctctaggactccagggtttatgctccaaagaacagaatttaccaggacaaaataaacaagaccagtcaggaccgatgccccatccctgctggggtctggcaaagctctcacctccaaatttgtatctgttttgaattcaaagccaaacaaacacatcaacagtgaactccaacacctcccagagcagggcctgaaagggacccagaaagtctggccagaaatctagagtccaaggggaggagatctgtaaactaaaccgctggccatgctctggggccctaaaccactgcaggcatcagggctgttccaggagagggcacagcaaagggggttgggaggggtctccagttccaatcagaaatgaggctgcagtcacttcaggtagacctgtcagcagcagctgtgcaactgggctagggagacaaggatcgtggtttagccaggagaatcatctggggccccagccaagacacaggtgttggatttcagcaccgctctgcaaatactcatctcagtgacgatgaggtgagtgggagcttggctgagcccagcccggcctgccatcctggcaagccagggcagcatggaggtagcacagagtggcacccagccagcgtgaatgcataagaatctgcacgtgacacagaagaaagtctcttcatgaagtaggtttcactggtcccagccaaaccctgtggcaggtggccctttctgcacctgctgaacatgccattcaccttgacccaggtagtggcctcaccctcctcttgctcaaactggaaacctcagcatcctgaaatgcctcctccccaaatccattgcacacatgtgtgcctgtgtatgcgtgtgtgtgcacgtgtatgaacccagcccccagctgcccactccattgcccctaaacaggcccctccttggtgtcacctggcacatctccactggaagccaaatggatatttctaaactgaaatctggtcccacctcagaaccccttccacagttcccttaaagttcctttcctcatttacatcaggatcttcacaatggggacccctggtcacctcccaacccaacaaacgctccaaatgagccgccactgcagaaactcattatggcccaggcaggacaggcacatccaagtatctgaccaggctgttccatctgccaggcaggtcctgccctctctccacccacctgtctaacccctgcatcctcaagaccctacttagctatggccctgtgtgaaaggtccctccccatgcacccacagccatttgttctctctcatgtggccctaacaggctggggttcctggagactccatggggagccaggcatgaagatggcatatacccatgtgtcactccccagaacgtgagctgcctgccctggcaccatacacaaagggactgacagccccagaatcccaaggggtgcacctatgcatatgggaaaggcatgtttacgggtgagaatggtccatcgttgggcttcaggaggcatctgacctgacgcacgcctttgtcactttgtccttgtggcctgttgaaatgccactcctgctttacaaattcaccaactgttgcatgagtcatttccacctcaatgagtaccaggtccttgaggatggggaaaagtaagccaccactgtgggggtcctgggctcctaggtgcagaagaggctccagaaacaggccaggtcgtgggccatgaccccacactagccctctggtccctcacacgggtggattggggggctgtgtcacgggatcttaggatcttcaagacaaagacccaggacaagaacacaagcccactcccattcttcacaggcctcgagaaatctttgggcaatgaagtcagactgtgccaaagcccatgtttctgtctctccaaggcccctggcccccactgcctagcctaggtcaggtcatgtgggcaagcgagcccccacagcctcacagcccctaccccagggccagggcaaactcctgccctgtccccctccattcctgccctccctccttccacaaactgcaccagctggggagaaatccttcagccgacagaatgaggtgaaaatagtgcaattttaggctttgtaactgagattagggcaggtggccacccattctccccttcctcaggccagcctctgacacaatgaccctggaagcctggcagccctccgtaatggtcagcatcctcccctgccatccccaacccacaccatgagctcagccagggcaggggcagcctctgtctcattcaccacagaatccacagaacccagcacagagtatgagctcagtaaattctcctcatacatgactgcactgactggaccgggcacatgctacagggcaacacccacggctcagctggccctggctttggatctcagtcccacctcttcaagctgtccagcgtggggcacatcggctacagccttgccaaatgaaggcttgccaggatgaagaggtgaagacaggacaagcacagtatgtggcacacaggaggcctctgataacatcagtccccttccctaaagacctgggcagtccctgtcactggggcctcacatttcatgtcgagaattcactatttctcagcactgatttcaaataaagccaccaagagtctgacgaggcaacatggcagagttctgagggtggagtgaacaaaaggtcattttttacagaaaactcaggatctcccctctgcacagtgctaaagccctgtctcaaagttcagagcccggaaggtgcagagatgtggcccttggaaatcaagcccttaagaaaacagcccagctgtgtagggccggaagccccaggctgcagtcctgtggtctggaggcagccaatattcaggtgagagatgtgcccagctgccggtgggtccagggggcacggagcccccaccgtccctggcccaggtctaggactaagtcagtgggcccaggccagctccaagggccacagctcctcactcgggggccgcgccggagcagccgcagcagctggggcgccgcagggactgcatgacagcccgcagtggccccctccggccctccacagacaggctgtcctcgctggcgggcgcccgctgcagctgctcaaactgcatctccaggtgcttctggatggccacaccgagcacctccaggtccaccgcagctccgtacacctcccatgtcatgccctcagcatcccatcgcacatcccgcacaggggacggcacctcctccaggctggaccccagagttacctctgggaacacatgcagggctgcaggcgcttccagggacggactggtggccacagccttgcaggccgccactggggccgcctgcacaccagcatcctgggctgacagcggggatgcctctgcaggggccaagtcattggctgaggtcatggtccacacatctttggtcctagagccaggctctgggactaacccagcgggaccccaaaggtgggcacagcaatgggaatgcccagggagccccccagacaacctacagtggatcttcaccccatgctgagcctgcagcccagactcgctcactgacgccactagtttgggaaaggccaggatccctgtggcaggtagggcatggcagcagccaccagccctcacctccctcatgccacagagtagagcagctgggggcagagcatggcaggtggtggtagccagctgttcagcagctttgggctcagcctgggcactgctgctgtgggcagttgtgtcccccaggtctagtggtggcactgacaactgactcgcccccagcatccaggctgagttagaagtctcatcctcaggagccaggtccctttccaggcctgcaggggcctggccaccctggccagaagtaccacctggctgcagctgagccctgtggacagggctgctgccaagggctgagcagctgagactggccttccgagcaccactgtgtccccgcatctgggtgctacggaccaggtctgaatggctcctctgcatagcagcagcactaggggcccgcaggcgacacaggtcactgccgcccatggtggacacattgcccacagtgctgctccaccagtggcctccagcactgggtcgcgccttggggccagaggcccgtgctggcttcatgctctcaggcgggttcccctcttcctccggggcctggggtctggtgctggcctcgcccagctgggcctgccacacggtgctgctggcagtcttgcggagctctggcctctgttcccggccttcacccagcaggctggaagagctctgggacaggggctgaaggcgggggctcaggggtgcccagggacccggctcggggcggctggagctcatggctgcctctagctccaggggcaaggagaggccccatgcatcagctttttccatgagggactcattcagcatctggtcattgattccacagcatctcctgagcccctactgcgtgcccagctgtagggctagggaacatgggattcattcagacctttctgtacccctgatgtgtcgtcggcactcagaggattatctgctgtgtgcctgaccaagagaacaagcaaatacaagaacacacccacagaggagggcactgagtgccaaaaatggggtctgagggagggcaccaccaaggcaggagagctcacggagggtgagagatgagaaaaggcttcctggaggaccagccacgtaagtcaggccttaatgttctctctcctgccccatttgatgccgaagttgctatggttgtggccgatgtcccgtggccaatgccaggctgtcctgctgcctcaggttccacctgtcagcaactctcaaggaccaggcaggaatgcacacagcacaaacccccattgcacagtggggatacagcaccctccaggaggtggtttaatccaccccagagtgaacggggcctgataggaacactcagggccaactctgggcaaagcagcaggcagcattccacgccccgcattgaggtctccgcgccggcggctacccctttcctctcgccttctccatcctagctccgcctctcac

SEQ ID NO: 15484 - RNA, 6820 nt, Homo sapiens
  source 1..6820: mol_type = other RNA
gctgggattacaggcatgagccactgtaccaggctgagtccacacttctaagcttgctgttgctctcagacttgcagaacaacctattaaacagaagtaggtaaaagttgagaaagggaagtggccaccacagaaccagttctgctgagaacgaggactcgagtcaggctatgctaccctccttccatggccatgggaaaaaggggtgtgtgctgttggtgtgagagatctggatcttaacagatcagacttaaactaatttgcccatgatgaccgtgtggatttggagggacctgggaatctcacagacctatgggatgtcccagtgatatgtcctgggcttcataccagccctgccctgcctgacaagttggatgaaaactgataaaggacttgtcatagcttcagatggcaaaaccaggccaggccagaatgaaaaaggagaaggaatttaacatgggcaaatgccaagctctgcatttaactaaccaaggctgcttggcgtgaacaaaactgagacagagcaatgcatggagaaaagggttgggcatttgtgggctacaagcttggcatgacatggatgcaaatgtcaatgggtgcacccccagatgcctgtgactccctctggtggtttctgtgcacaacttcccccaaaataggccctacgactccagcagaaacctaccctggggctcctagagcttcctagcctgcctgccagagagcagaagtgcctggaggctacatcttcacccctgggtagtccttactctgaggtgggactgcatccagggctcccctttagggtctgacttggactgaaatcacaccctgccttgccttctgcccctcccttaacttgctctcccctccctaataactccagcatcctcatctcagcagaagcttctggggaacccagcccaagatgagtggtgagggctagggtagccctcctcaatgcactctgggaactacattttcagaagccccagccagagggccaagtcccaggcagggtgcaaagctgtggggcgaggaacctggaaagaggctctgaacaagggacttttaaggaagtgggatgtgggctgtgatcacagccaagctggcagggtaagaggtggcccctgaatgtggctatgagaggggtgcccaacactaccagcctgtgtgctgagcactaactcagtgccaggcactacttgggttattctatttaatctccacaccaagcatgtgaaggaggcaccattgtcatccccatcttacagatgaggaagatgatcaaggcttgtaacttgcccaagatcacatggctataggtgtggatcctatatatccagattcaaactccagctttagcccactaagctacggtggccaaccccagcccaaagtgttgggacctgcgtgtagaagaccccttcagcccttgtaaagttaggatctagcatgtctaaggggacagagacccaatccaggtgacacaggaggtaagatcacagtggaacaggccatccctgcttttccaccaccaccagcactgtgacctcagaccagctctactctatgagtttcttgtgacagtgatggcagcctggggccagacaagggatgcgtgtcttgtgtcctggacacaagacaggcaggcccagaggggacaagctatatgaagagaggcttcagctgtcgggggtcctgaatgccatggaaggagagcaggtgggcagaagcagggagcccctggagcagacagaggggggattcctgctgaggcaaggggctctaggactccagggtttatgctccaaagaacagaatttaccaggacaaaataaacaagaccagtcaggaccgatgccccatccctgctggggtctggcaaagctctcacctccaaatttgtatctgttttgaattcaaagccaaacaaacacatcaacagtgaactccaacacctcccagagcagggcctgaaagggacccagaaagtctggccagaaatctagagtccaaggggaggagatctgtaaactaaaccgctggccatgctctggggccctaaaccactgcaggcatcagggctgttccaggagagggcacagcaaagggggttgggaggggtctccagttccaatcagaaatgaggctgcagtcacttcaggtagacctgtcagcagcagctgtgcaactgggctagggagacaaggatcgtggtttagccaggagaatcatctggggccccagccaagacacaggtgttggatttcagcaccgctctgcaaatactcatctcagtgacgatgaggtgagtgggagcttggctgagcccagcccggcctgccatcctggcaagccagggcagcatggaggtagcacagagtggcacccagccagcgtgaatgcataagaatctgcacgtgacacagaagaaagtctcttcatgaagtaggtttcactggtcccagccaaaccctgtggcaggtggccctttctgcacctgctgaacatgccattcaccttgacccaggtagtggcctcaccctcctcttgctcaaactggaaacctcagcatcctgaaatgcctcctccccaaatccattgcacacatgtgtgcctgtgtatgcgtgtgtgtgcacgtgtatgaacccagcccccagctgcccactccattgcccctaaacaggcccctccttggtgtcacctggcacatctccactggaagccaaatggatatttctaaactgaaatctggtcccacctcagaaccccttccacagttcccttaaagttcctttcctcatttacatcaggatcttcacaatggggacccctggtcacctcccaacccaacaaacgctccaaatgagccgccactgcagaaactcattatggcccaggcaggacaggcacatccaagtatctgaccaggctgttccatctgccaggcaggtcctgccctctctccacccacctgtctaacccctgcatcctcaagaccctacttagctatggccctgtgtgaaaggtccctccccatgcacccacagccatttgttctctctcatgtggccctaacaggctggggttcctggagactccatggggagccaggcatgaagatggcatatacccatgtgtcactccccagaacgtgagctgcctgccctggcaccatacacaaagggactgacagccccagaatcccaaggggtgcacctatgcatatgggaaaggcatgtttacgggtgagaatggtccatcgttgggcttcaggaggcatctgacctgacgcacgcctttgtcactttgtccttgtggcctgttgaaatgccactcctgctttacaaattcaccaactgttgcatgagtcatttccacctcaatgagtaccaggtccttgaggatggggaaaagtaagccaccactgtgggggtcctgggctcctaggtgcagaagaggctccagaaacaggccaggtcgtgggccatgaccccacactagccctctggtccctcacacgggtggattggggggctgtgtcacgggatcttaggatcttcaagacaaagacccaggacaagaacacaagcccactcccattcttcacaggcctcgagaaatctttgggcaatgaagtcagactgtgccaaagcccatgtttctgtctctccaaggcccctggcccccactgcctagcctaggtcaggtcatgtgggcaagcgagcccccacagcctcacagcccctaccccagggccagggcaaactcctgccctgtccccctccattcctgccctccctccttccacaaactgcaccagctggggagaaatccttcagccgacagaatgaggtgaaaatagtgcaattttaggctttgtaactgagattagggcaggtggccacccattctccccttcctcaggccagcctctgacacaatgaccctggaagcctggcagccctccgtaatggtcagcatcctcccctgccatccccaacccacaccatgagctcagccagggcaggggcagcctctgtctcattcaccacagaatccacagaacccagcacagagtatgagctcagtaaattctcctcatacatgactgcactgactggaccgggcacatgctacagggcaacacccacggctcagctggccctggctttggatctcagtcccacctcttcaagctgtccagcgtggggcacatcggctacagccttgccaaatgaaggcttgccaggatgaagaggtgaagacaggacaagcacagtatgtggcacacaggaggcctctgataacatcagtccccttccctaaagacctgggcagtccctgtcactggggcctcacatttcatgtcgagaattcactatttctcagcactgatttcaaataaagccaccaagagtctgacgaggcaacatggcagagttctgagggtggagtgaacaaaaggtcattttttacagaaaactcaggatctcccctctgcacagtgctaaagccctgtctcaaagttcagagcccggaaggtgcagagatgtggcccttggaaatcaagcccttaagaaaacagcccagctgtgtagggccggaagccccaggctgcagtcctgtggtctggaggcagccaatattcaggtgagagatgtgcccagctgccggtgggtccagggggcacggagcccccaccgtccctggcccaggtctaggactaagtcagtgggcccaggccagctccaagggccacagctcctcactcgggggccgcgccggagcagccgcagcagctggggcgccgcagggactgcatgacagcccgcagtggccccctccggccctccacagacaggctgtcctcgctggcgggcgcccgctgcagctgctcaaactgcatctccaggtgcttctggatggccacaccgagcacctccaggtccaccgcagctccgtacacctcccatgtcatgccctcagcatcccatcgcacatcccgcacaggggacggcacctcctccaggctggaccccagagttacctctgggaacacatgcagggctgcaggcgcttccagggacggactggtggccacagccttgcaggccgccactggggccgcctgcacaccagcatcctgggctgacagcggggatgcctctgcaggggccaagtcattggctgaggtcatggtccacacatctttggtcctagagccaggctctgggactaacccagcgggaccccaaaggtgggcacagcaatgggaatgcccagggagccccccagacaacctacagtggatcttcaccccatgctgagcctgcagcccagactcgctcactgacgccactagtttgggaaaggccaggatccctgtggcaggtagggcatggcagcagccaccagccctcacctccctcatgccacagagtagagcagctgggggcagagcatggcaggtggtggtagccagctgttcagcagctttgggctcagcctgggcactgctgctgtgggcagttgtgtcccccaggtctagtggtggcactgacaactgactcgcccccagcatccaggctgagttagaagtctcatcctcaggagccaggtccctttccaggcctgcaggggcctggccaccctggccagaagtaccacctggctgcagctgagccctgtggacagggctgctgccaagggctgagcagctgagactggccttccgagcaccactgtgtccccgcatctgggtgctacggaccaggtctgaatggctcctctgcatagcagcagcactaggggcccgcaggcgacacaggtcactgccgcccatggtggacacattgcccacagtgctgctccaccagtggcctccagcactgggtcgcgccttggggccagaggcccgtgctggcttcatgctctcaggcgggttcccctcttcctccggggcctggggtctggtgctggcctcgcccagctgggcctgccacacggtgctgctggcagtcttgcggagctctggcctctgttcccggccttcacccagcaggctggaagagctctgggacaggggctgaaggcgggggctcaggggtgcccagggacccggctcggggcggctggagctcatggctgcctctagctccaggggcaaggagaggccccatgcatcagctttttccatgagggactcattcagcatctggtcattgattccacagcatctcctgagcccctactgcgtgcccagctgtagggctagggaacatgggattcattcagacctttctgtacccctgatgtgtcgtcggcactcagaggattatctgctgtgtgcctgaccaagagaacaagcaaatacaagaacacacccacagaggagggcactgagtgccaaaaatggggtctgagggagggcaccaccaaggcaggagagctcacggagggtgagagatgagaaaaggcttcctggaggaccagccacgtaagtcaggccttaatgttctctctcctgccccatttgatgccgaagttgctatggttgtggccgatgtcccgtggccaatgccaggctgtcctgctgcctcaggttccacctgtcagcaactctcaaggaccaggcaggaatgcacacagcacaaacccccattgcacagtggggatacagcaccctccaggaggtggtttaatccaccccagagtgaacggggcctgataggaacactcagggccaactctgggcaaagcagcaggcagcattcccctttcctctcgccttctccatcctagctccgcctctcac

SEQ ID NO: 15485 - RNA, 6919 nt, Homo sapiens
  source 1..6919: mol_type = other RNA
gctgggattacaggcatgagccactgtaccaggctgagtccacacttctaagcttgctgttgctctcagacttgcagaacaacctattaaacagaagtaggtaaaagttgagaaagggaagtggccaccacagaaccagttctgctgagaacgaggactcgagtcaggctatgctaccctccttccatggccatgggaaaaaggggtgtgtgctgttggtgtgagagatctggatcttaacagatcagacttaaactaatttgcccatgatgaccgtgtggatttggagggacctgggaatctcacagacctatgggatgtcccagtgatatgtcctgggcttcataccagccctgccctgcctgacaagttggatgaaaactgataaaggacttgtcatagcttcagatggcaaaaccaggccaggccagaatgaaaaaggagaaggaatttaacatgggcaaatgccaagctctgcatttaactaaccaaggctgcttggcgtgaacaaaactgagacagagcaatgcatggagaaaagggttgggcatttgtgggctacaagcttggcatgacatggatgcaaatgtcaatgggtgcacccccagatgcctgtgactccctctggtggtttctgtgcacaacttcccccaaaataggccctacgactccagcagaaacctaccctggggctcctagagcttcctagcctgcctgccagagagcagaagtgcctggaggctacatcttcacccctgggtagtccttactctgaggtgggactgcatccagggctcccctttagggtctgacttggactgaaatcacaccctgccttgccttctgcccctcccttaacttgctctcccctccctaataactccagcatcctcatctcagcagaagcttctggggaacccagcccaagatgagtggtgagggctagggtagccctcctcaatgcactctgggaactacattttcagaagccccagccagagggccaagtcccaggcagggtgcaaagctgtggggcgaggaacctggaaagaggctctgaacaagggacttttaaggaagtgggatgtgggctgtgatcacagccaagctggcagggtaagaggtggcccctgaatgtggctatgagaggggtgcccaacactaccagcctgtgtgctgagcactaactcagtgccaggcactacttgggttattctatttaatctccacaccaagcatgtgaaggaggcaccattgtcatccccatcttacagatgaggaagatgatcaaggcttgtaacttgcccaagatcacatggctataggtgtggatcctatatatccagattcaaactccagctttagcccactaagctacggtggccaaccccagcccaaagtgttgggacctgcgtgtagaagaccccttcagcccttgtaaagttaggatctagcatgtctaaggggacagagacccaatccaggtgacacaggaggtaagatcacagtggaacaggccatccctgcttttccaccaccaccagcactgtgacctcagaccagctctactctatgagtttcttgtgacagtgatggcagcctggggccagacaagggatgcgtgtcttgtgtcctggacacaagacaggcaggcccagaggggacaagctatatgaagagaggcttcagctgtcgggggtcctgaatgccatggaaggagagcaggtgggcagaagcagggagcccctggagcagacagaggggggattcctgctgaggcaaggggctctaggactccagggtttatgctccaaagaacagaatttaccaggacaaaataaacaagaccagtcaggaccgatgccccatccctgctggggtctggcaaagctctcacctccaaatttgtatctgttttgaattcaaagccaaacaaacacatcaacagtgaactccaacacctcccagagcagggcctgaaagggacccagaaagtctggccagaaatctagagtccaaggggaggagatctgtaaactaaaccgctggccatgctctggggccctaaaccactgcaggcatcagggctgttccaggagagggcacagcaaagggggttgggaggggtctccagttccaatcagaaatgaggctgcagtcacttcaggtagacctgtcagcagcagctgtgcaactgggctagggagacaaggatcgtggtttagccaggagaatcatctggggccccagccaagacacaggtgttggatttcagcaccgctctgcaaatactcatctcagtgacgatgaggtgagtgggagcttggctgagcccagcccggcctgccatcctggcaagccagggcagcatggaggtagcacagagtggcacccagccagcgtgaatgcataagaatctgcacgtgacacagaagaaagtctcttcatgaagtaggtttcactggtcccagccaaaccctgtggcaggtggccctttctgcacctgctgaacatgccattcaccttgacccaggtagtggcctcaccctcctcttgctcaaactggaaacctcagcatcctgaaatgcctcctccccaaatccattgcacacatgtgtgcctgtgtatgcgtgtgtgtgcacgtgtatgaacccagcccccagctgcccactccattgcccctaaacaggcccctccttggtgtcacctggcacatctccactggaagccaaatggatatttctaaactgaaatctggtcccacctcagaaccccttccacagttcccttaaagttcctttcctcatttacatcaggatcttcacaatggggacccctggtcacctcccaacccaacaaacgctccaaatgagccgccactgcagaaactcattatggcccaggcaggacaggcacatccaagtatctgaccaggctgttccatctgccaggcaggtcctgccctctctccacccacctgtctaacccctgcatcctcaagaccctacttagctatggccctgtgtgaaaggtccctccccatgcacccacagccatttgttctctctcatgtggccctaacaggctggggttcctggagactccatggggagccaggcatgaagatggcatatacccatgtgtcactccccagaacgtgagctgcctgccctggcaccatacacaaagggactgacagccccagaatcccaaggggtgcacctatgcatatgggaaaggcatgtttacgggtgagaatggtccatcgttgggcttcaggaggcatctgacctgacgcacgcctttgtcactttgtccttgtggcctgttgaaatgccactcctgctttacaaattcaccaactgttgcatgagtcatttccacctcaatgagtaccaggtccttgaggatggggaaaagtaagccaccactgtgggggtcctgggctcctaggtgcagaagaggctccagaaacaggccaggtcgtgggccatgaccccacactagccctctggtccctcacacgggtggattggggggctgtgtcacgggatcttaggatcttcaagacaaagacccaggacaagaacacaagcccactcccattcttcacaggcctcgagaaatctttgggcaatgaagtcagactgtgccaaagcccatgtttctgtctctccaaggcccctggcccccactgcctagcctaggtcaggtcatgtgggcaagcgagcccccacagcctcacagcccctaccccagggccagggcaaactcctgccctgtccccctccattcctgccctccctccttccacaaactgcaccagctggggagaaatccttcagccgacagaatgaggtgaaaatagtgcaattttaggctttgtaactgagattagggcaggtggccacccattctccccttcctcaggccagcctctgacacaatgaccctggaagcctggcagccctccgtaatggtcagcatcctcccctgccatccccaacccacaccatgagctcagccagggcaggggcagcctctgtctcattcaccacagaatccacagaacccagcacagagtatgagctcagtaaattctcctcatacatgactgcactgactggaccgggcacatgctacagggcaacacccacggctcagctggccctggctttggatctcagtcccacctcttcaagctgtccagcgtggggcacatcggctacagccttgccaaatgaaggcttgccaggatgaagaggtgaagacaggacaagcacagtatgtggcacacaggaggcctctgataacatcagtccccttccctaaagacctgggcagtccctgtcactggggcctcacatttcatgtcgagaattcactatttctcagcactgatttcaaataaagccaccaagagtctgacgaggcaacatggcagagttctgagggtggagtgaacaaaaggtcattttttacagaaaactcaggatctcccctctgcacagtgctaaagccctgtctcaaagttcagagcccggaaggtgcagagatgtggcccttggaaatcaagcccttaagaaaacagcccagctgtgtagggccggaagccccaggctgcagtcctgtggtctggaggcagccaatattcaggtgagagatgtgcccagctgccggtgggtccagggggcacggagcccccaccgtccctggcccaggtctaggactaagtcagtgggcccaggccagctccaagggccacagctcctcactcgggggccgcgccggagcagccgcagcagctggggcgccgcagggactgcatgacagcccgcagtggccccctccggccctccacagacaggctgtcctcgctggcgggcgcccgctgcagctgctcaaactgcatctccaggtgcttctggatggccacaccgagcacctccaggtccaccgcagctccgtacacctcccatgtcatgccctcagcatcccatcgcacatcccgcacaggggacggcacctcctccaggctggaccccagagttacctctgggaacacatgcagggctgcaggcgcttccagggacggactggtggccacagccttgcaggccgccactggggccgcctgcacaccagcatcctgggctgacagcggggatgcctctgcaggggccaagtcattggctgaggtcatggtccacacatctttggtcctagagccaggctctgggactaacccagcgggaccccaaaggtgggcacagcaatgggaatgcccagggagccccccagacaacctacagtggatcttcaccccatgctgagcctgcagcccagactcgctcactgacgccactagtttgggaaaggccaggatccctgtggcaggtagggcatggcagcagccaccagccctcacctccctcatgccacagagtagagcagctgggggcagagcatggcaggtggtggtagccagctgttcagcagctttgggctcagcctgggcactgctgctgtgggcagttgtgtcccccaggtctagtggtggcactgacaactgactcgcccccagcatccaggctgagttagaagtctcatcctcaggagccaggtccctttccaggcctgcaggggcctggccaccctggccagaagtaccacctggctgcagctgagccctgtggacagggctgctgccaagggctgagcagctgagactggccttccgagcaccactgtgtccccgcatctgggtgctacggaccaggtctgaatggctcctctgcatagcagcagcactaggggcccgcaggcgacacaggtcactgccgcccatggtggacacattgcccacagtgctgctccaccagtggcctccagcactgggtcgcgccttggggccagaggcccgtgctggcttcatgctctcaggcgggttcccctcttcctccggggcctggggtctggtgctggcctcgcccagctgggcctgccacacggtgctgctggcagtcttgcggagctctggcctctgttcccggccttcacccagcaggctggaagagctctgggacaggggctgaaggcgggggctcaggggtgcccagggacccggctcggggcggctggagctcatggctgcctctagctccaggggcaaggagaggccccatgcatcagctttttccatgagggactcattcagcatctggtcattgattccacagcatctcctgagcccctactgcgtgcccagctgtagggctagggaacatgggattcattcagacctttctgtacccctgatgtgtcgtcggcactcagaggattatctgctgtgtgcctgaccaagagaacaagcaaatacaagaacacacccacagaggagggcactgagtgccaaaaatggggtctgagggagggcaccaccaaggcaggagagctcacggagggtgagagatgagaaaaggcttcctggaggaccagccacgtaagtcaggccttaatgttctctctcctgccccatttgatgccgaagttgctatggttgtggccgatgtcccgtggccaatgccaggctgtcctgctgcctcaggttccacctgtcagcaactctcaaggaccaggcaggaatgcacacagcacaaacccccattgcacagtggggatacagcaccctccaggaggtggtttaatccaccccagagtgaacggggcctgataggaacactcagggccaactctgggcaaagcagcaggcagcattccctctcgcccgccggggccgcgcaggcgggggaagcgctgctcctgcggccgccacaggtgccaggtgccgcggcccaagatggagccagagccgacctggcctgggcgcgagacgccgcccgccgccgtcggcccggcc

SEQ ID NO: 15486 - RNA, 6502 nt, Homo sapiens
  source 1..6502: mol_type = other RNA
gctgggattacaggcatgagccactgtaccaggctgagtccacacttctaagcttgctgttgctctcagacttgcagaacaacctattaaacagaagtaggtaaaagttgagaaagggaagtggccaccacagaaccagttctgctgagaacgaggactcgagtcaggctatgctaccctccttccatggccatgggaaaaaggggtgtgtgctgttggtgtgagagatctggatcttaacagatcagacttaaactaatttgcccatgatgaccgtgtggatttggagggacctgggaatctcacagacctatgggatgtcccagtgatatgtcctgggcttcataccagccctgccctgcctgacaagttggatgaaaactgataaaggacttgtcatagcttcagatggcaaaaccaggccaggccagaatgaaaaaggagaaggaatttaacatgggcaaatgccaagctctgcatttaactaaccaaggctgcttggcgtgaacaaaactgagacagagcaatgcatggagaaaagggttgggcatttgtgggctacaagcttggcatgacatggatgcaaatgtcaatgggtgcacccccagatgcctgtgactccctctggtggtttctgtgcacaacttcccccaaaataggccctacgactccagcagaaacctaccctggggctcctagagcttcctagcctgcctgccagagagcagaagtgcctggaggctacatcttcacccctgggtagtccttactctgaggtgggactgcatccagggctcccctttagggtctgacttggactgaaatcacaccctgccttgccttctgcccctcccttaacttgctctcccctccctaataactccagcatcctcatctcagcagaagcttctggggaacccagcccaagatgagtggtgagggctagggtagccctcctcaatgcactctgggaactacattttcagaagccccagccagagggccaagtcccaggcagggtgcaaagctgtggggcgaggaacctggaaagaggctctgaacaagggacttttaaggaagtgggatgtgggctgtgatcacagccaagctggcagggtaagaggtggcccctgaatgtggctatgagaggggtgcccaacactaccagcctgtgtgctgagcactaactcagtgccaggcactacttgggttattctatttaatctccacaccaagcatgtgaaggaggcaccattgtcatccccatcttacagatgaggaagatgatcaaggcttgtaacttgcccaagatcacatggctataggtgtggatcctatatatccagattcaaactccagctttagcccactaagctacggtggccaaccccagcccaaagtgttgggacctgcgtgtagaagaccccttcagcccttgtaaagttaggatctagcatgtctaaggggacagagacccaatccaggtgacacaggaggtaagatcacagtggaacaggccatccctgcttttccaccaccaccagcactgtgacctcagaccagctctactctatgagtttcttgtgacagtgatggcagcctggggccagacaagggatgcgtgtcttgtgtcctggacacaagacaggcaggcccagaggggacaagctatatgaagagaggcttcagctgtcgggggtcctgaatgccatggaaggagagcaggtgggcagaagcagggagcccctggagcagacagaggggggattcctgctgaggcaaggggctctaggactccagggtttatgctccaaagaacagaatttaccaggacaaaataaacaagaccagtcaggaccgatgccccatccctgctggggtctggcaaagctctcacctccaaatttgtatctgttttgaattcaaagccaaacaaacacatcaacagtgaactccaacacctcccagagcagggcctgaaagggacccagaaagtctggccagaaatctagagtccaaggggaggagatctgtaaactaaaccgctggccatgctctggggccctaaaccactgcaggcatcagggctgttccaggagagggcacagcaaagggggttgggaggggtctccagttccaatcagaaatgaggctgcagtcacttcaggtagacctgtcagcagcagctgtgcaactgggctagggagacaaggatcgtggtttagccaggagaatcatctggggccccagccaagacacaggtgttggatttcagcaccgctctgcaaatactcatctcagtgacgatgaggtgagtgggagcttggctgagcccagcccggcctgccatcctggcaagccagggcagcatggaggtagcacagagtggcacccagccagcgtgaatgcataagaatctgcacgtgacacagaagaaagtctcttcatgaagtaggtttcactggtcccagccaaaccctgtggcaggtggccctttctgcacctgctgaacatgccattcaccttgacccaggtagtggcctcaccctcctcttgctcaaactggaaacctcagcatcctgaaatgcctcctccccaaatccattgcacacatgtgtgcctgtgtatgcgtgtgtgtgcacgtgtatgaacccagcccccagctgcccactccattgcccctaaacaggcccctccttggtgtcacctggcacatctccactggaagccaaatggatatttctaaactgaaatctggtcccacctcagaaccccttccacagttcccttaaagttcctttcctcatttacatcaggatcttcacaatggggacccctggtcacctcccaacccaacaaacgctccaaatgagccgccactgcagaaactcattatggcccaggcaggacaggcacatccaagtatctgaccaggctgttccatctgccaggcaggtcctgccctctctccacccacctgtctaacccctgcatcctcaagaccctacttagctatggccctgtgtgaaaggtccctccccatgcacccacagccatttgttctctctcatgtggccctaacaggctggggttcctggagactccatggggagccaggcatgaagatggcatatacccatgtgtcactccccagaacgtgagctgcctgccctggcaccatacacaaagggactgacagccccagaatcccaaggggtgcacctatgcatatgggaaaggcatgtttacgggtgagaatggtccatcgttgggcttcaggaggcatctgacctgacgcacgcctttgtcactttgtccttgtggcctgttgaaatgccactcctgctttacaaattcaccaactgttgcatgagtcatttccacctcaatgagtaccaggtccttgaggatggggaaaagtaagccaccactgtgggggtcctgggctcctaggtgcagaagaggctccagaaacaggccaggtcgtgggccatgaccccacactagccctctggtccctcacacgggtggattggggggctgtgtcacgggatcttaggatcttcaagacaaagacccaggacaagaacacaagcccactcccattcttcacaggcctcgagaaatctttgggcaatgaagtcagactgtgccaaagcccatgtttctgtctctccaaggcccctggcccccactgcctagcctaggtcaggtcatgtgggcaagcgagcccccacagcctcacagcccctaccccagggccagggcaaactcctgccctgtccccctccattcctgccctccctccttccacaaactgcaccagctggggagaaatccttcagccgacagaatgaggtgaaaatagtgcaattttaggctttgtaactgagattagggcaggtggccacccattctccccttcctcaggccagcctctgacacaatgaccctggaagcctggcagccctccgtaatggtcagcatcctcccctgccatccccaacccacaccatgagctcagccagggcaggggcagcctctgtctcattcaccacagaatccacagaacccagcacagagtatgagctcagtaaattctcctcatacatgactgcactgactggaccgggcacatgctacagggcaacacccacggctcagctggccctggctttggatctcagtcccacctcttcaagctgtccagcgtggggcacatcggctacagccttgccaaatgaaggcttgccaggatgaagaggtgaagacaggacaagcacagtatgtggcacacaggaggcctctgataacatcagtccccttccctaaagacctgggcagtccctgtcactggggcctcacatttcatgtcgagaattcactatttctcagcactgatttcaaataaagccaccaagagtctgacgaggcaacatggcagagttctgagggtggagtgaacaaaaggtcattttttacagaaaactcaggatctcccctctgcacagtgctaaagccctgtctcaaagttcagagcccggaaggtgcagagatgtggcccttggaaatcaagcccttaagaaaacagcccagctgtgtagggccggaagccccaggctgcagtcctgtggtctggaggcagccaatattcaggtgagagatgtgcccagctgccggtgggtccagggggcacggagcccccaccgtccctggcccaggtctaggactaagtcagtgggcccaggccagctccaagggccacagctcctcactcgggggccgcgccggagcagccgcagcagctggggcgccgcagggactgcatgacagcccgcagtggccccctccggccctccacagacaggctgtcctcgctggcgggcgcccgctgcagctgctcaaactgcatctccaggtgcttctggatggccacaccgagcacctccaggtccaccgcagctccgtacacctcccatgtcatgccctcagcatcccatcgcacatcccgcacaggggacggcacctcctccaggctggaccccagagttacctctgggaacacatgcagggctgcaggcgcttccagggacggactggtggccacagccttgcaggccgccactggggccgcctgcacaccagcatcctgggctgacagcggggatgcctctgcaggggccaagtcattggctgaggtcatggtccacacatctttggtcctagagccaggctctgggactaacccagcgggaccccaaaggtgggcacagcaatgggaatgcccagggagccccccagacaacctacagtggatcttcaccccatgctgagcctgcagcccagactcgctcactgacgccactagtttgggaaaggccaggatccctgtggcaggtagggcatggcagcagccaccagccctcacctccctcatgccacagagtagagcagctgggggcagagcatggcaggtggtggtagccagctgttcagcagctttgggctcagcctgggcactgctgctgtgggcagttgtgtcccccaggtctagtggtggcactgacaactgactcgcccccagcatccaggctgagttagaagtctcatcctcaggagccaggtccctttccaggcctgcaggggcctggccaccctggccagaagtaccacctggctgcagctgagccctgtggacagggctgctgccaagggctgagcagctgagactggccttccgagcaccactgtgtccccgcatctgggtgctacggaccaggtctgaatggctcctctgcatagcagcagcactaggggcccgcaggcgacacaggtcactgccgcccatggtggacacattgcccacagtgctgctccaccagtggcctccagcactgggtcgcgccttggggccagaggcccgtgctggcttcatgctctcaggcgggttcccctcttcctccggggcctggggtctggtgctggcctcgcccagctgggcctgccacacggtgctgctggcagtcttgcggagctctggcctctgttcccggccttcacccagcaggctggaagagctctgggacaggggctgaaggcgggggctcaggggtgcccagggacccggctcggggcggctggagctcatggctgcctctagctccaggggcaaggagaggccccatgcatcagctttttccatgagggactcattcagcatctggtcattgattccacagcatctcctgagcccctactgcgtgcccagctgtagggctagggaacatgggattcattcagacctttctgtaccccttaatgttctctctcctgccccatttgatgccgaagttgctatggttgtggccgatgtcccgtggccaatgccaggctgtcctgctgcctcaggttccacctgtcagcaacacgccccgcattgaggtctccgcgccggcggctacccctttcctctcgccttctccatcctagctccgcctctcac

SEQ ID NO: 15487 - RNA, 6554 nt, Homo sapiens
  source 1..6554: mol_type = other RNA
gctgggattacaggcatgagccactgtaccaggctgagtccacacttctaagcttgctgttgctctcagacttgcagaacaacctattaaacagaagtaggtaaaagttgagaaagggaagtggccaccacagaaccagttctgctgagaacgaggactcgagtcaggctatgctaccctccttccatggccatgggaaaaaggggtgtgtgctgttggtgtgagagatctggatcttaacagatcagacttaaactaatttgcccatgatgaccgtgtggatttggagggacctgggaatctcacagacctatgggatgtcccagtgatatgtcctgggcttcataccagccctgccctgcctgacaagttggatgaaaactgataaaggacttgtcatagcttcagatggcaaaaccaggccaggccagaatgaaaaaggagaaggaatttaacatgggcaaatgccaagctctgcatttaactaaccaaggctgcttggcgtgaacaaaactgagacagagcaatgcatggagaaaagggttgggcatttgtgggctacaagcttggcatgacatggatgcaaatgtcaatgggtgcacccccagatgcctgtgactccctctggtggtttctgtgcacaacttcccccaaaataggccctacgactccagcagaaacctaccctggggctcctagagcttcctagcctgcctgccagagagcagaagtgcctggaggctacatcttcacccctgggtagtccttactctgaggtgggactgcatccagggctcccctttagggtctgacttggactgaaatcacaccctgccttgccttctgcccctcccttaacttgctctcccctccctaataactccagcatcctcatctcagcagaagcttctggggaacccagcccaagatgagtggtgagggctagggtagccctcctcaatgcactctgggaactacattttcagaagccccagccagagggccaagtcccaggcagggtgcaaagctgtggggcgaggaacctggaaagaggctctgaacaagggacttttaaggaagtgggatgtgggctgtgatcacagccaagctggcagggtaagaggtggcccctgaatgtggctatgagaggggtgcccaacactaccagcctgtgtgctgagcactaactcagtgccaggcactacttgggttattctatttaatctccacaccaagcatgtgaaggaggcaccattgtcatccccatcttacagatgaggaagatgatcaaggcttgtaacttgcccaagatcacatggctataggtgtggatcctatatatccagattcaaactccagctttagcccactaagctacggtggccaaccccagcccaaagtgttgggacctgcgtgtagaagaccccttcagcccttgtaaagttaggatctagcatgtctaaggggacagagacccaatccaggtgacacaggaggtaagatcacagtggaacaggccatccctgcttttccaccaccaccagcactgtgacctcagaccagctctactctatgagtttcttgtgacagtgatggcagcctggggccagacaagggatgcgtgtcttgtgtcctggacacaagacaggcaggcccagaggggacaagctatatgaagagaggcttcagctgtcgggggtcctgaatgccatggaaggagagcaggtgggcagaagcagggagcccctggagcagacagaggggggattcctgctgaggcaaggggctctaggactccagggtttatgctccaaagaacagaatttaccaggacaaaataaacaagaccagtcaggaccgatgccccatccctgctggggtctggcaaagctctcacctccaaatttgtatctgttttgaattcaaagccaaacaaacacatcaacagtgaactccaacacctcccagagcagggcctgaaagggacccagaaagtctggccagaaatctagagtccaaggggaggagatctgtaaactaaaccgctggccatgctctggggccctaaaccactgcaggcatcagggctgttccaggagagggcacagcaaagggggttgggaggggtctccagttccaatcagaaatgaggctgcagtcacttcaggtagacctgtcagcagcagctgtgcaactgggctagggagacaaggatcgtggtttagccaggagaatcatctggggccccagccaagacacaggtgttggatttcagcaccgctctgcaaatactcatctcagtgacgatgaggtgagtgggagcttggctgagcccagcccggcctgccatcctggcaagccagggcagcatggaggtagcacagagtggcacccagccagcgtgaatgcataagaatctgcacgtgacacagaagaaagtctcttcatgaagtaggtttcactggtcccagccaaaccctgtggcaggtggccctttctgcacctgctgaacatgccattcaccttgacccaggtagtggcctcaccctcctcttgctcaaactggaaacctcagcatcctgaaatgcctcctccccaaatccattgcacacatgtgtgcctgtgtatgcgtgtgtgtgcacgtgtatgaacccagcccccagctgcccactccattgcccctaaacaggcccctccttggtgtcacctggcacatctccactggaagccaaatggatatttctaaactgaaatctggtcccacctcagaaccccttccacagttcccttaaagttcctttcctcatttacatcaggatcttcacaatggggacccctggtcacctcccaacccaacaaacgctccaaatgagccgccactgcagaaactcattatggcccaggcaggacaggcacatccaagtatctgaccaggctgttccatctgccaggcaggtcctgccctctctccacccacctgtctaacccctgcatcctcaagaccctacttagctatggccctgtgtgaaaggtccctccccatgcacccacagccatttgttctctctcatgtggccctaacaggctggggttcctggagactccatggggagccaggcatgaagatggcatatacccatgtgtcactccccagaacgtgagctgcctgccctggcaccatacacaaagggactgacagccccagaatcccaaggggtgcacctatgcatatgggaaaggcatgtttacgggtgagaatggtccatcgttgggcttcaggaggcatctgacctgacgcacgcctttgtcactttgtccttgtggcctgttgaaatgccactcctgctttacaaattcaccaactgttgcatgagtcatttccacctcaatgagtaccaggtccttgaggatggggaaaagtaagccaccactgtgggggtcctgggctcctaggtgcagaagaggctccagaaacaggccaggtcgtgggccatgaccccacactagccctctggtccctcacacgggtggattggggggctgtgtcacgggatcttaggatcttcaagacaaagacccaggacaagaacacaagcccactcccattcttcacaggcctcgagaaatctttgggcaatgaagtcagactgtgccaaagcccatgtttctgtctctccaaggcccctggcccccactgcctagcctaggtcaggtcatgtgggcaagcgagcccccacagcctcacagcccctaccccagggccagggcaaactcctgccctgtccccctccattcctgccctccctccttccacaaactgcaccagctggggagaaatccttcagccgacagaatgaggtgaaaatagtgcaattttaggctttgtaactgagattagggcaggtggccacccattctccccttcctcaggccagcctctgacacaatgaccctggaagcctggcagccctccgtaatggtcagcatcctcccctgccatccccaacccacaccatgagctcagccagggcaggggcagcctctgtctcattcaccacagaatccacagaacccagcacagagtatgagctcagtaaattctcctcatacatgactgcactgactggaccgggcacatgctacagggcaacacccacggctcagctggccctggctttggatctcagtcccacctcttcaagctgtccagcgtggggcacatcggctacagccttgccaaatgaaggcttgccaggatgaagaggtgaagacaggacaagcacagtatgtggcacacaggaggcctctgataacatcagtccccttccctaaagacctgggcagtccctgtcactggggcctcacatttcatgtcgagaattcactatttctcagcactgatttcaaataaagccaccaagagtctgacgaggcaacatggcagagttctgagggtggagtgaacaaaaggtcattttttacagaaaactcaggatctcccctctgcacagtgctaaagccctgtctcaaagttcagagcccggaaggtgcagagatgtggcccttggaaatcaagcccttaagaaaacagcccagctgtgtagggccggaagccccaggctgcagtcctgtggtctggaggcagccaatattcaggtgagagatgtgcccagctgccggtgggtccagggggcacggagcccccaccgtccctggcccaggtctaggactaagtcagtgggcccaggccagctccaagggccacagctcctcactcgggggccgcgccggagcagccgcagcagctggggcgccgcagggactgcatgacagcccgcagtggccccctccggccctccacagacaggctgtcctcgctggcgggcgcccgctgcagctgctcaaactgcatctccaggtgcttctggatggccacaccgagcacctccaggtccaccgcagctccgtacacctcccatgtcatgccctcagcatcccatcgcacatcccgcacaggggacggcacctcctccaggctggaccccagagttacctctgggaacacatgcagggctgcaggcgcttccagggacggactggtggccacagccttgcaggccgccactggggccgcctgcacaccagcatcctgggctgacagcggggatgcctctgcaggggccaagtcattggctgaggtcatggtccacacatctttggtcctagagccaggctctgggactaacccagcgggaccccaaaggtgggcacagcaatgggaatgcccagggagccccccagacaacctacagtggatcttcaccccatgctgagcctgcagcccagactcgctcactgacgccactagtttgggaaaggccaggatccctgtggcaggtagggcatggcagcagccaccagccctcacctccctcatgccacagagtagagcagctgggggcagagcatggcaggtggtggtagccagctgttcagcagctttgggctcagcctgggcactgctgctgtgggcagttgtgtcccccaggtctagtggtggcactgacaactgactcgcccccagcatccaggctgagttagaagtctcatcctcaggagccaggtccctttccaggcctgcaggggcctggccaccctggccagaagtaccacctggctgcagctgagccctgtggacagggctgctgccaagggctgagcagctgagactggccttccgagcaccactgtgtccccgcatctgggtgctacggaccaggtctgaatggctcctctgcatagcagcagcactaggggcccgcaggcgacacaggtcactgccgcccatggtggacacattgcccacagtgctgctccaccagtggcctccagcactgggtcgcgccttggggccagaggcccgtgctggcttcatgctctcaggcgggttcccctcttcctccggggcctggggtctggtgctggcctcgcccagctgggcctgccacacggtgctgctggcagtcttgcggagctctggcctctgttcccggccttcacccagcaggctggaagagctctgggacaggggctgaaggcgggggctcaggggtgcccagggacccggctcggggcggctggagctcatggctgcctctagctccaggggcaaggagaggccccatgcatcagctttttccatgagggactcattcagcatctggtcattgattccacagcatctcctgagcccctactgcgtgcccagctgtagggctagggaacatgggattcattcagacctttctgtaccccttaatgttctctctcctgccccatttgatgccgaagttgctatggttgtggccgatgtcccgtggccaatgccaggctgtcctgctgcctcaggttccacctgtcagcaaccagcccgacttgaggccttcagtctcccagccgcggaccccaacagcgggcgagggcagtgaccgtgcggggatgagccacctccactggagcccgccttcttctccgcaattccccgcagcaccaca

SEQ ID NO: 15488 - RNA, 7092 nt, Homo sapiens
  source 1..7092: mol_type = other RNA
gctgggattacaggcatgagccactgtaccaggctgagtccacacttctaagcttgctgttgctctcagacttgcagaacaacctattaaacagaagtaggtaaaagttgagaaagggaagtggccaccacagaaccagttctgctgagaacgaggactcgagtcaggctatgctaccctccttccatggccatgggaaaaaggggtgtgtgctgttggtgtgagagatctggatcttaacagatcagacttaaactaatttgcccatgatgaccgtgtggatttggagggacctgggaatctcacagacctatgggatgtcccagtgatatgtcctgggcttcataccagccctgccctgcctgacaagttggatgaaaactgataaaggacttgtcatagcttcagatggcaaaaccaggccaggccagaatgaaaaaggagaaggaatttaacatgggcaaatgccaagctctgcatttaactaaccaaggctgcttggcgtgaacaaaactgagacagagcaatgcatggagaaaagggttgggcatttgtgggctacaagcttggcatgacatggatgcaaatgtcaatgggtgcacccccagatgcctgtgactccctctggtggtttctgtgcacaacttcccccaaaataggccctacgactccagcagaaacctaccctggggctcctagagcttcctagcctgcctgccagagagcagaagtgcctggaggctacatcttcacccctgggtagtccttactctgaggtgggactgcatccagggctcccctttagggtctgacttggactgaaatcacaccctgccttgccttctgcccctcccttaacttgctctcccctccctaataactccagcatcctcatctcagcagaagcttctggggaacccagcccaagatgagtggtgagggctagggtagccctcctcaatgcactctgggaactacattttcagaagccccagccagagggccaagtcccaggcagggtgcaaagctgtggggcgaggaacctggaaagaggctctgaacaagggacttttaaggaagtgggatgtgggctgtgatcacagccaagctggcagggtaagaggtggcccctgaatgtggctatgagaggggtgcccaacactaccagcctgtgtgctgagcactaactcagtgccaggcactacttgggttattctatttaatctccacaccaagcatgtgaaggaggcaccattgtcatccccatcttacagatgaggaagatgatcaaggcttgtaacttgcccaagatcacatggctataggtgtggatcctatatatccagattcaaactccagctttagcccactaagctacggtggccaaccccagcccaaagtgttgggacctgcgtgtagaagaccccttcagcccttgtaaagttaggatctagcatgtctaaggggacagagacccaatccaggtgacacaggaggtaagatcacagtggaacaggccatccctgcttttccaccaccaccagcactgtgacctcagaccagctctactctatgagtttcttgtgacagtgatggcagcctggggccagacaagggatgcgtgtcttgtgtcctggacacaagacaggcaggcccagaggggacaagctatatgaagagaggcttcagctgtcgggggtcctgaatgccatggaaggagagcaggtgggcagaagcagggagcccctggagcagacagaggggggattcctgctgaggcaaggggctctaggactccagggtttatgctccaaagaacagaatttaccaggacaaaataaacaagaccagtcaggaccgatgccccatccctgctggggtctggcaaagctctcacctccaaatttgtatctgttttgaattcaaagccaaacaaacacatcaacagtgaactccaacacctcccagagcagggcctgaaagggacccagaaagtctggccagaaatctagagtccaaggggaggagatctgtaaactaaaccgctggccatgctctggggccctaaaccactgcaggcatcagggctgttccaggagagggcacagcaaagggggttgggaggggtctccagttccaatcagaaatgaggctgcagtcacttcaggtagacctgtcagcagcagctgtgcaactgggctagggagacaaggatcgtggtttagccaggagaatcatctggggccccagccaagacacaggtgttggatttcagcaccgctctgcaaatactcatctcagtgacgatgaggtgagtgggagcttggctgagcccagcccggcctgccatcctggcaagccagggcagcatggaggtagcacagagtggcacccagccagcgtgaatgcataagaatctgcacgtgacacagaagaaagtctcttcatgaagtaggtttcactggtcccagccaaaccctgtggcaggtggccctttctgcacctgctgaacatgccattcaccttgacccaggtagtggcctcaccctcctcttgctcaaactggaaacctcagcatcctgaaatgcctcctccccaaatccattgcacacatgtgtgcctgtgtatgcgtgtgtgtgcacgtgtatgaacccagcccccagctgcccactccattgcccctaaacaggcccctccttggtgtcacctggcacatctccactggaagccaaatggatatttctaaactgaaatctggtcccacctcagaaccccttccacagttcccttaaagttcctttcctcatttacatcaggatcttcacaatggggacccctggtcacctcccaacccaacaaacgctccaaatgagccgccactgcagaaactcattatggcccaggcaggacaggcacatccaagtatctgaccaggctgttccatctgccaggcaggtcctgccctctctccacccacctgtctaacccctgcatcctcaagaccctacttagctatggccctgtgtgaaaggtccctccccatgcacccacagccatttgttctctctcatgtggccctaacaggctggggttcctggagactccatggggagccaggcatgaagatggcatatacccatgtgtcactccccagaacgtgagctgcctgccctggcaccatacacaaagggactgacagccccagaatcccaaggggtgcacctatgcatatgggaaaggcatgtttacgggtgagaatggtccatcgttgggcttcaggaggcatctgacctgacgcacgcctttgtcactttgtccttgtggcctgttgaaatgccactcctgctttacaaattcaccaactgttgcatgagtcatttccacctcaatgagtaccaggtccttgaggatggggaaaagtaagccaccactgtgggggtcctgggctcctaggtgcagaagaggctccagaaacaggccaggtcgtgggccatgaccccacactagccctctggtccctcacacgggtggattggggggctgtgtcacgggatcttaggatcttcaagacaaagacccaggacaagaacacaagcccactcccattcttcacaggcctcgagaaatctttgggcaatgaagtcagactgtgccaaagcccatgtttctgtctctccaaggcccctggcccccactgcctagcctaggtcaggtcatgtgggcaagcgagcccccacagcctcacagcccctaccccagggccagggcaaactcctgccctgtccccctccattcctgccctccctccttccacaaactgcaccagctggggagaaatccttcagccgacagaatgaggtgaaaatagtgcaattttaggctttgtaactgagattagggcaggtggccacccattctccccttcctcaggccagcctctgacacaatgaccctggaagcctggcagccctccgtaatggtcagcatcctcccctgccatccccaacccacaccatgagctcagccagggcaggggcagcctctgtctcattcaccacagaatccacagaacccagcacagagtatgagctcagtaaattctcctcatacatgactgcactgactggaccgggcacatgctacagggcaacacccacggctcagctggccctggctttggatctcagtcccacctcttcaagctgtccagcgtggggcacatcggctacagccttgccaaatgaaggcttgccaggatgaagaggtgaagacaggacaagcacagtatgtggcacacaggaggcctctgataacatcagtccccttccctaaagacctgggcagtccctgtcactggggcctcacatttcatgtcgagaattcactatttctcagcactgatttcaaataaagccaccaagagtctgacgaggcaacatggcagagttctgagggtggagtgaacaaaaggtcattttttacagaaaactcaggatctcccctctgcacagtgctaaagccctgtctcaaagttcagagcccggaaggtgcagagatgtggcccttggaaatcaagcccttaagaaaacagcccagctgtgtagggccggaagccccaggctgcagtcctgtggtctggaggcagccaatattcaggtgagagatgtgcccagctgccggtgggtccagggggcacggagcccccaccgtccctggcccaggtctaggactaagtcagtgggcccaggccagctccaagggccacagctcctcactcgggggccgcgccggagcagccgcagcagctggggcgccgcagggactgcatgacagcccgcagtggccccctccggccctccacagacaggctgtcctcgctggcgggcgcccgctgcagctgctcaaactgcatctccaggtgcttctggatggccacaccgagcacctccaggtccaccgcagctccgtacacctcccatgtcatgccctcagcatcccatcgcacatcccgcacaggggacggcacctcctccaggctggaccccagagttacctctgggaacacatgcagggctgcaggcgcttccagggacggactggtggccacagccttgcaggccgccactggggccgcctgcacaccagcatcctgggctgacagcggggatgcctctgcaggggccaagtcattggctgaggtcatggtccacacatctttggtcctagagccaggctctgggactaacccagcgggaccccaaaggtgggcacagcaatgggaatgcccagggagccccccagacaacctacagtggatcttcaccccatgctgagcctgcagcccagactcgctcactgacgccactagtttgggaaaggccaggatccctgtggcaggtagggcatggcagcagccaccagccctcacctccctcatgccacagagtagagcagctgggggcagagcatggcaggtggtggtagccagctgttcagcagctttgggctcagcctgggcactgctgctgtgggcagttgtgtcccccaggtctagtggtggcactgacaactgactcgcccccagcatccaggctgagttagaagtctcatcctcaggagccaggtccctttccaggcctgcaggggcctggccaccctggccagaagtaccacctggctgcagctgagccctgtggacagggctgctgccaagggctgagcagctgagactggccttccgagcaccactgtgtccccgcatctgggtgctacggaccaggtctgaatggctcctctgcatagcagcagcactaggggcccgcaggcgacacaggtcactgccgcccatggtggacacattgcccacagtgctgctccaccagtggcctccagcactgggtcgcgccttggggccagaggcccgtgctggcttcatgctctcaggcgggttcccctcttcctccggggcctggggtctggtgctggcctcgcccagctgggcctgccacacggtgctgctggcagtcttgcggagctctggcctctgttcccggccttcacccagcaggctggaagagctctgggacaggggctgaaggcgggggctcaggggtgcccagggacccggctcggggcggctggagctcatggctgcctctagctccaggggcaaggagaggccccatgcatcagctttttccatgagggactcattcagcatctggtcattgattccacagcatctcctgagcccctactgcgtgcccagctgtagggctagggaacatgggattcattcagacctttctgtaccccttaatgttctctctcctgccccatttgatgccgaagttgctatggttgtggccgatgtcccgtggccaatgccaggctgtcctgctgcctcaggttccacctgtcagcaactctcaaggaccaggcaggaatgcacacagcacaaacccccattgcacagtggggatacagcaccctccaggaggtggtttaatccaccccagagtgaacggggcctgataggaacactcagggccaactctgggcaaagcagcaggcagcattcctaaagggagggtttggaggagacaaaacctgcccttcacaatgaacgtgccttaagggctacatgccccgggtcacaagctgtgccaggaaagggttctggggtaactgtggggtcagtggccccatggatgaggctctgctcaccaggaagaggcctaggcgcccaacagcccctgagcttcctcccctggggaggatttgcccacaatccctggggggcacctaggtggagagggtgccccggcctagaagcagcctaggcggccggtgtgtccctatctgcacgctcacaagcactcatgccccagcctgggacacacaggcccgtatgcagtaacagcgtctacccagctgcactctgcacgccaagcacaggccgcccctgctgcggggccaaaggcctgaaagcaccgcaccacgcagcctcgcccagaatagctcccctcccgcccctcctgcacaaagcccacccggacttagggagaagggggctcaatacgggcccgaaac

SEQ ID NO: 15489 - RNA, 9158 nt, Homo sapiens
  source 1..9158: mol_type = other RNA
gctgggattacaggcatgagccactgtaccaggctgagtccacacttctaagcttgctgttgctctcagacttgcagaacaacctattaaacagaagtaggtaaaagttgagaaagggaagtggccaccacagaaccagttctgctgagaacgaggactcgagtcaggctatgctaccctccttccatggccatgggaaaaaggggtgtgtgctgttggtgtgagagatctggatcttaacagatcagacttaaactaatttgcccatgatgaccgtgtggatttggagggacctgggaatctcacagacctatgggatgtcccagtgatatgtcctgggcttcataccagccctgccctgcctgacaagttggatgaaaactgataaaggacttgtcatagcttcagatggcaaaaccaggccaggccagaatgaaaaaggagaaggaatttaacatgggcaaatgccaagctctgcatttaactaaccaaggctgcttggcgtgaacaaaactgagacagagcaatgcatggagaaaagggttgggcatttgtgggctacaagcttggcatgacatggatgcaaatgtcaatgggtgcacccccagatgcctgtgactccctctggtggtttctgtgcacaacttcccccaaaataggccctacgactccagcagaaacctaccctggggctcctagagcttcctagcctgcctgccagagagcagaagtgcctggaggctacatcttcacccctgggtagtccttactctgaggtgggactgcatccagggctcccctttagggtctgacttggactgaaatcacaccctgccttgccttctgcccctcccttaacttgctctcccctccctaataactccagcatcctcatctcagcagaagcttctggggaacccagcccaagatgagtggtgagggctagggtagccctcctcaatgcactctgggaactacattttcagaagccccagccagagggccaagtcccaggcagggtgcaaagctgtggggcgaggaacctggaaagaggctctgaacaagggacttttaaggaagtgggatgtgggctgtgatcacagccaagctggcagggtaagaggtggcccctgaatgtggctatgagaggggtgcccaacactaccagcctgtgtgctgagcactaactcagtgccaggcactacttgggttattctatttaatctccacaccaagcatgtgaaggaggcaccattgtcatccccatcttacagatgaggaagatgatcaaggcttgtaacttgcccaagatcacatggctataggtgtggatcctatatatccagattcaaactccagctttagcccactaagctacggtggccaaccccagcccaaagtgttgggacctgcgtgtagaagaccccttcagcccttgtaaagttaggatctagcatgtctaaggggacagagacccaatccaggtgacacaggaggtaagatcacagtggaacaggccatccctgcttttccaccaccaccagcactgtgacctcagaccagctctactctatgagtttcttgtgacagtgatggcagcctggggccagacaagggatgcgtgtcttgtgtcctggacacaagacaggcaggcccagaggggacaagctatatgaagagaggcttcagctgtcgggggtcctgaatgccatggaaggagagcaggtgggcagaagcagggagcccctggagcagacagaggggggattcctgctgaggcaaggggctctaggactccagggtttatgctccaaagaacagaatttaccaggacaaaataaacaagaccagtcaggaccgatgccccatccctgctggggtctggcaaagctctcacctccaaatttgtatctgttttgaattcaaagccaaacaaacacatcaacagtgaactccaacacctcccagagcagggcctgaaagggacccagaaagtctggccagaaatctagagtccaaggggaggagatctgtaaactaaaccgctggccatgctctggggccctaaaccactgcaggcatcagggctgttccaggagagggcacagcaaagggggttgggaggggtctccagttccaatcagaaatgaggctgcagtcacttcaggtagacctgtcagcagcagctgtgcaactgggctagggagacaaggatcgtggtttagccaggagaatcatctggggccccagccaagacacaggtgttggatttcagcaccgctctgcaaatactcatctcagtgacgatgaggtgagtgggagcttggctgagcccagcccggcctgccatcctggcaagccagggcagcatggaggtagcacagagtggcacccagccagcgtgaatgcataagaatctgcacgtgacacagaagaaagtctcttcatgaagtaggtttcactggtcccagccaaaccctgtggcaggtggccctttctgcacctgctgaacatgccattcaccttgacccaggtagtggcctcaccctcctcttgctcaaactggaaacctcagcatcctgaaatgcctcctccccaaatccattgcacacatgtgtgcctgtgtatgcgtgtgtgtgcacgtgtatgaacccagcccccagctgcccactccattgcccctaaacaggcccctccttggtgtcacctggcacatctccactggaagccaaatggatatttctaaactgaaatctggtcccacctcagaaccccttccacagttcccttaaagttcctttcctcatttacatcaggatcttcacaatggggacccctggtcacctcccaacccaacaaacgctccaaatgagccgccactgcagaaactcattatggcccaggcaggacaggcacatccaagtatctgaccaggctgttccatctgccaggcaggtcctgccctctctccacccacctgtctaacccctgcatcctcaagaccctacttagctatggccctgtgtgaaaggtccctccccatgcacccacagccatttgttctctctcatgtggccctaacaggctggggttcctggagactccatggggagccaggcatgaagatggcatatacccatgtgtcactccccagaacgtgagctgcctgccctggcaccatacacaaagggactgacagccccagaatcccaaggggtgcacctatgcatatgggaaaggcatgtttacgggtgagaatggtccatcgttgggcttcaggaggcatctgacctgacgcacgcctttgtcactttgtccttgtggcctgttgaaatgccactcctgctttacaaattcaccaactgttgcatgagtcatttccacctcaatgagtaccaggtccttgaggatggggaaaagtaagccaccactgtgggggtcctgggctcctaggtgcagaagaggctccagaaacaggccaggtcgtgggccatgaccccacactagccctctggtccctcacacgggtggattggggggctgtgtcacgggatcttaggatcttcaagacaaagacccaggacaagaacacaagcccactcccattcttcacaggcctcgagaaatctttgggcaatgaagtcagactgtgccaaagcccatgtttctgtctctccaaggcccctggcccccactgcctagcctaggtcaggtcatgtgggcaagcgagcccccacagcctcacagcccctaccccagggccagggcaaactcctgccctgtccccctccattcctgccctccctccttccacaaactgcaccagctggggagaaatccttcagccgacagaatgaggtgaaaatagtgcaattttaggctttgtaactgagattagggcaggtggccacccattctccccttcctcaggccagcctctgacacaatgaccctggaagcctggcagccctccgtaatggtcagcatcctcccctgccatccccaacccacaccatgagctcagccagggcaggggcagcctctgtctcattcaccacagaatccacagaacccagcacagagtatgagctcagtaaattctcctcatacatgactgcactgactggaccgggcacatgctacagggcaacacccacggctcagctggccctggctttggatctcagtcccacctcttcaagctgtccagcgtggggcacatcggctacagccttgccaaatgaaggcttgccaggatgaagaggtgaagacaggacaagcacagtatgtggcacacaggaggcctctgataacatcagtccccttccctaaagacctgggcagtccctgtcactggggcctcacatttcatgtcgagaattcactatttctcagcactgatttcaaataaagccaccaagagtctgacgaggcaacatggcagagttctgagggtggagtgaacaaaaggtcattttttacagaaaactcaggatctcccctctgcacagtgctaaagccctgtctcaaagttcagagcccggaaggtgcagagatgtggcccttggaaatcaagcccttaagaaaacagcccagctgtgtagggccggaagccccaggctgcagtcctgtggtctggaggcagccaatattcaggtgagagatgtgcccagctgccggtgggtccagggggcacggagcccccaccgtccctggcccaggtctaggactaagtcagtgggcccaggccagctccaagggccacagctcctcactcgggggccgcgccggagcagccgcagcagctggggcgccgcagggactgcatgacagcccgcagtggccccctccggccctccacagacaggctgtcctcgctggcgggcgcccgctgcagctgctcaaactgcatctccaggtgcttctggatggccacaccgagcacctccaggtccaccgcagctccgtacacctcccatgtcatgccctcagcatcccatcgcacatcccgcacaggggacggcacctcctccaggctggaccccagagttacctctgggaacacatgcagggctgcaggcgcttccagggacggactggtggccacagccttgcaggccgccactggggccgcctgcacaccagcatcctgggctgacagcggggatgcctctgcaggggccaagtcattggctgaggtcatggtccacacatctttggtcctagagccaggctctgggactaacccagcgggaccccaaaggtgggcacagcaatgggaatgcccagggagccccccagacaacctacagtggatcttcaccccatgctgagcctgcagcccagactcgctcactgacgccactagtttgggaaaggccaggatccctgtggcaggtagggcatggcagcagccaccagccctcacctccctcatgccacagagtagagcagctgggggcagagcatggcaggtggtggtagccagctgttcagcagctttgggctcagcctgggcactgctgctgtgggcagttgtgtcccccaggtctagtggtggcactgacaactgactcgcccccagcatccaggctgagttagaagtctcatcctcaggagccaggtccctttccaggcctgcaggggcctggccaccctggccagaagtaccacctggctgcagctgagccctgtggacagggctgctgccaagggctgagcagctgagactggccttccgagcaccactgtgtccccgcatctgggtgctacggaccaggtctgaatggctcctctgcatagcagcagcactaggggcccgcaggcgacacaggtcactgccgcccatggtggacacattgcccacagtgctgctccaccagtggcctccagcactgggtcgcgccttggggccagaggcccgtgctggcttcatgctctcaggcgggttcccctcttcctccggggcctggggtctggtgctggcctcgcccagctgggcctgccacacggtgctgctggcagtcttgcggagctctggcctctgttcccggccttcacccagcaggctggaagagctctgggacaggggctgaaggcgggggctcaggggtgcccagggacccggctcggggcggctggagctcatggctgcctctagctccaggggcaaggagaggccccatgcatcagctttttccatgagggactcattcagcatctggtcattgattccacagcatctcctgagcccctactgcgtgcccagctgtagggctgatgtgtcgtcggcactcagaggattatctgctgtgtgcctgaccaagagaacaagcaaatacaagaacacacccacagaggagggcactgagtgccaaaaatggggtctgagggagggcaccaccaaggcaggagagctcacggagggtgagagatgagaaaaggcttcctggaggaccagccacgtaagtcaggcctggagtgagagaagcaagaaggtgttcaggtggagagcggagtgggcaggaggaaagaggccatgtgtccagagcatatgaggggagcagtggggtcaaagtgtctgggccacctcggccctggccacagcagtgaattagggagatcactctgggactccttgccaggcaggagaggtgggagaaacagggtggggacaggaggcagcagctgcatttgggcaatcccagccctgccctcccagcctaggctgataaagacttccaggcaacaacctccccgaccaggtgagcaaggctacccgagaggaaattcgggaagggctgtgggactcggtttctgtgtaattacaaatgtcctggcagcccagcactcaggagatggctggtggctgctgagccacagtgaggatgatactggtgctgtagtccctgagactccagctctgcacaacttcctgcgatgatggaaagattctaccctgtgctgtccaataggtaggcaccaatggcatgtgggtaccaagcactcagcagggggctactgcaactgagacactgaatgtttaagttttatttgaatctaactggccacatgaggctaatggctaccgtacaggactgtgcagctctgaacacagccccggcctggtaaggatgtcccatcccagctgcttcacggggctgaagccagacttgtccctgggaggatcaggaagaggaggagtagccaagagagaaatctgacccagaccctgccctcaatgagctctaagatggacatacaaacaaaggagggcaataaagcccgtaacagcgatgataataacagctgccagggcctgatcactcgccaagggccagacacgtgccacatcctttgcatacattgtctcatataactgtgcaagcaacctcttgagacagtcattatctccattctacagacaggagaattccataagctcagagaggctcagtgacccccaagggcacacacctgtggggcagctgagctcctctccccttcgagcactgagcaggcctatgcctcgcagctctcaccctttttactgatctggcctggccctgccaatcgtgctcatgacatgccatggaacaagtcactgagtggatctccacctgcccaacatgcttcttagcagctcctgaggctgcaagaatgaggagggcaggaggtgttcctcctgactgggacagctgtggtcactgccagcccctggcagggagacaaccactcagttgcaggtccaagaccccagggaggccccatctggacatccacacagcctctggccaaaccccaccaccctcccagggaggggggccataaacagccaggccagcagcctctggcccctgaggagacaggtggaatgaggtcctcagacccccaccaagacccactgagaagccatgagcaatgagcatcccactgtgcctgtctcaccagagggctgcccagcacccagggctagtcatcacccagagacccccgtgtgggctatgtatctattggttcccttccccattccccctccacaagtggcaggtgacaaaactgaggcctggagcagctcagaaatgtcaaagaacacacagctgaaagtggctaattcagaaccccaatggattggcctggctaactacaacctggccttcccagctcagaaggaaggaagggctctgaggggagtactgggggaaagaggcttccacactgcctgtcacagtgctgtggactgggccagaggaggggcctcccagggagccaggggtgaggaggaaggggcagggctctgcttccaatgggggctcttccccttcctgtgcatgtactcacaggtggacccctaacttctttgagcctcagtttcttcaatcttaatgttctctctcctgccccatttgatgccgaagttgctatggttgtggccgatgtcccgtggccaatgccaggctgtcctgctgcctcaggttccacctgtcagcaactctcaaggaccaggcaggaatgcacacagcacaaacccccattgcacagtggggatacagcaccctccaggaggtggtttaatccaccccagagtgaacggggcctgataggaacactcagggccaactctgggcaaagcagcaggcagcattcctaaagggagggtttggaggagacaaaacctgcccttcacaatgaacgtgccttaagggctacatgccccgggtcacaagctgtgccaggaaagggttctggggtaactgtggggtcagtggccccatggatgaggctctgctcaccaggaagaggcctaggcgcccaacagcccctgagcttcctcccctggggaggatttgcccacaatccctggggggcacctaggtggagagggtgccccggcctagaagcagcctaggcggccggtgtgtccctatctgcacgctcacaagcactcatgccccagcctgggacacacaggcccgtatgcagtaacagcgtctacccagctgcactctgcacgccaagcacaggccgcccctgctgcggggccaaaggcctgaaagcaccgcaccacgcagcctcgcccagaatagctcccctcccgcccctcctgcacaaagcccacccggacttagggagaagggggctcaatacgggcccgaaac

SEQ ID NO: 15490 - RNA, 6663 nt, Homo sapiens
  source 1..6663: mol_type = other RNA
gctgggattacaggcatgagccactgtaccaggctgagtccacacttctaagcttgctgttgctctcagacttgcagaacaacctattaaacagaagtaggtaaaagttgagaaagggaagtggccaccacagaaccagttctgctgagaacgaggactcgagtcaggctatgctaccctccttccatggccatgggaaaaaggggtgtgtgctgttggtgtgagagatctggatcttaacagatcagacttaaactaatttgcccatgatgaccgtgtggatttggagggacctgggaatctcacagacctatgggatgtcccagtgatatgtcctgggcttcataccagccctgccctgcctgacaagttggatgaaaactgataaaggacttgtcatagcttcagatggcaaaaccaggccaggccagaatgaaaaaggagaaggaatttaacatgggcaaatgccaagctctgcatttaactaaccaaggctgcttggcgtgaacaaaactgagacagagcaatgcatggagaaaagggttgggcatttgtgggctacaagcttggcatgacatggatgcaaatgtcaatgggtgcacccccagatgcctgtgactccctctggtggtttctgtgcacaacttcccccaaaataggccctacgactccagcagaaacctaccctggggctcctagagcttcctagcctgcctgccagagagcagaagtgcctggaggctacatcttcacccctgggtagtccttactctgaggtgggactgcatccagggctcccctttagggtctgacttggactgaaatcacaccctgccttgccttctgcccctcccttaacttgctctcccctccctaataactccagcatcctcatctcagcagaagcttctggggaacccagcccaagatgagtggtgagggctagggtagccctcctcaatgcactctgggaactacattttcagaagccccagccagagggccaagtcccaggcagggtgcaaagctgtggggcgaggaacctggaaagaggctctgaacaagggacttttaaggaagtgggatgtgggctgtgatcacagccaagctggcagggtaagaggtggcccctgaatgtggctatgagaggggtgcccaacactaccagcctgtgtgctgagcactaactcagtgccaggcactacttgggttattctatttaatctccacaccaagcatgtgaaggaggcaccattgtcatccccatcttacagatgaggaagatgatcaaggcttgtaacttgcccaagatcacatggctataggtgtggatcctatatatccagattcaaactccagctttagcccactaagctacggtggccaaccccagcccaaagtgttgggacctgcgtgtagaagaccccttcagcccttgtaaagttaggatctagcatgtctaaggggacagagacccaatccaggtgacacaggaggtaagatcacagtggaacaggccatccctgcttttccaccaccaccagcactgtgacctcagaccagctctactctatgagtttcttgtgacagtgatggcagcctggggccagacaagggatgcgtgtcttgtgtcctggacacaagacaggcaggcccagaggggacaagctatatgaagagaggcttcagctgtcgggggtcctgaatgccatggaaggagagcaggtgggcagaagcagggagcccctggagcagacagaggggggattcctgctgaggcaaggggctctaggactccagggtttatgctccaaagaacagaatttaccaggacaaaataaacaagaccagtcaggaccgatgccccatccctgctggggtctggcaaagctctcacctccaaatttgtatctgttttgaattcaaagccaaacaaacacatcaacagtgaactccaacacctcccagagcagggcctgaaagggacccagaaagtctggccagaaatctagagtccaaggggaggagatctgtaaactaaaccgctggccatgctctggggccctaaaccactgcaggcatcagggctgttccaggagagggcacagcaaagggggttgggaggggtctccagttccaatcagaaatgaggctgcagtcacttcaggtagacctgtcagcagcagctgtgcaactgggctagggagacaaggatcgtggtttagccaggagaatcatctggggccccagccaagacacaggtgttggatttcagcaccgctctgcaaatactcatctcagtgacgatgaggtgagtgggagcttggctgagcccagcccggcctgccatcctggcaagccagggcagcatggaggtagcacagagtggcacccagccagcgtgaatgcataagaatctgcacgtgacacagaagaaagtctcttcatgaagtaggtttcactggtcccagccaaaccctgtggcaggtggccctttctgcacctgctgaacatgccattcaccttgacccaggtagtggcctcaccctcctcttgctcaaactggaaacctcagcatcctgaaatgcctcctccccaaatccattgcacacatgtgtgcctgtgtatgcgtgtgtgtgcacgtgtatgaacccagcccccagctgcccactccattgcccctaaacaggcccctccttggtgtcacctggcacatctccactggaagccaaatggatatttctaaactgaaatctggtcccacctcagaaccccttccacagttcccttaaagttcctttcctcatttacatcaggatcttcacaatggggacccctggtcacctcccaacccaacaaacgctccaaatgagccgccactgcagaaactcattatggcccaggcaggacaggcacatccaagtatctgaccaggctgttccatctgccaggcaggtcctgccctctctccacccacctgtctaacccctgcatcctcaagaccctacttagctatggccctgtgtgaaaggtccctccccatgcacccacagccatttgttctctctcatgtggccctaacaggctggggttcctggagactccatggggagccaggcatgaagatggcatatacccatgtgtcactccccagaacgtgagctgcctgccctggcaccatacacaaagggactgacagccccagaatcccaaggggtgcacctatgcatatgggaaaggcatgtttacgggtgagaatggtccatcgttgggcttcaggaggcatctgacctgacgcacgcctttgtcactttgtccttgtggcctgttgaaatgccactcctgctttacaaattcaccaactgttgcatgagtcatttccacctcaatgagtaccaggtccttgaggatggggaaaagtaagccaccactgtgggggtcctgggctcctaggtgcagaagaggctccagaaacaggccaggtcgtgggccatgaccccacactagccctctggtccctcacacgggtggattggggggctgtgtcacgggatcttaggatcttcaagacaaagacccaggacaagaacacaagcccactcccattcttcacaggcctcgagaaatctttgggcaatgaagtcagactgtgccaaagcccatgtttctgtctctccaaggcccctggcccccactgcctagcctaggtcaggtcatgtgggcaagcgagcccccacagcctcacagcccctaccccagggccagggcaaactcctgccctgtccccctccattcctgccctccctccttccacaaactgcaccagctggggagaaatccttcagccgacagaatgaggtgaaaatagtgcaattttaggctttgtaactgagattagggcaggtggccacccattctccccttcctcaggccagcctctgacacaatgaccctggaagcctggcagccctccgtaatggtcagcatcctcccctgccatccccaacccacaccatgagctcagccagggcaggggcagcctctgtctcattcaccacagaatccacagaacccagcacagagtatgagctcagtaaattctcctcatacatgactgcactgactggaccgggcacatgctacagggcaacacccacggctcagctggccctggctttggatctcagtcccacctcttcaagctgtccagcgtggggcacatcggctacagccttgccaaatgaaggcttgccaggatgaagaggtgaagacaggacaagcacagtatgtggcacacaggaggcctctgataacatcagtccccttccctaaagacctgggcagtccctgtcactggggcctcacatttcatgtcgagaattcactatttctcagcactgatttcaaataaagccaccaagagtctgacgaggcaacatggcagagttctgagggtggagtgaacaaaaggtcattttttacagaaaactcaggatctcccctctgcacagtgctaaagccctgtctcaaagttcagagcccggaaggtgcagagatgtggcccttggaaatcaagcccttaagaaaacagcccagctgtgtagggccggaagccccaggctgcagtcctgtggtctggaggcagccaatattcaggtgagagatgtgcccagctgccggtgggtccagggggcacggagcccccaccgtccctggcccaggtctaggactaagtcagtgggcccaggccagctccaagggccacagctcctcactcgggggccgcgccggagcagccgcagcagctggggcgccgcagggactgcatgacagcccgcagtggccccctccggccctccacagacaggctgtcctcgctggcgggcgcccgctgcagctgctcaaactgcatctccaggtgcttctggatggccacaccgagcacctccaggtccaccgcagctccgtacacctcccatgtcatgccctcagcatcccatcgcacatcccgcacaggggacggcacctcctccaggctggaccccagagttacctctgggaacacatgcagggctgcaggcgcttccagggacggactggtggccacagccttgcaggccgccactggggccgcctgcacaccagcatcctgggctgacagcggggatgcctctgcaggggccaagtcattggctgaggtcatggtccacacatctttggtcctagagccaggctctgggactaacccagcgggaccccaaaggtgggcacagcaatgggaatgcccagggagccccccagacaacctacagtggatcttcaccccatgctgagcctgcagcccagactcgctcactgacgccactagtttgggaaaggccaggatccctgtggcaggtagggcatggcagcagccaccagccctcacctccctcatgccacagagtagagcagctgggggcagagcatggcaggtggtggtagccagctgttcagcagctttgggctcagcctgggcactgctgctgtgggcagttgtgtcccccaggtctagtggtggcactgacaactgactcgcccccagcatccaggctgagttagaagtctcatcctcaggagccaggtccctttccaggcctgcaggggcctggccaccctggccagaagtaccacctggctgcagctgagccctgtggacagggctgctgccaagggctgagcagctgagactggccttccgagcaccactgtgtccccgcatctgggtgctacggaccaggtctgaatggctcctctgcatagcagcagcactaggggcccgcaggcgacacaggtcactgccgcccatggtggacacattgcccacagtgctgctccaccagtggcctccagcactgggtcgcgccttggggccagaggcccgtgctggcttcatgctctcaggcgggttcccctcttcctccggggcctggggtctggtgctggcctcgcccagctgggcctgccacacggtgctgctggcagtcttgcggagctctggcctctgttcccggccttcacccagcaggctggaagagctctgggacaggggctgaaggcgggggctcaggggtgcccagggacccggctcggggcggctggagctcatggctgcctctagctccaggggcaaggagaggccccatgcatcagctttttccatgagggactcattcagcatctggtcattgattccacagcatctcctgagcccctactgcgtgcccagctgtagggctgatgtgtcgtcggcactcagaggattatctgctgtgtgcctgaccaagagaacaagcaaatacaagaacacacccacagaggagggcactgagtgccaaaaatggggtctgagggagggcaccaccaaggcaggagagctcacggagggtgagagatgagaaaaggcttcctggaggaccagccacgtaagtcaggccttaatgttctctctcctgccccatttgatgccgaagttgctatggttgtggccgatgtcccgtggccaatgccaggctgtcctgctgcctcaggttccacctgtcagcaacacgccccgcattgaggtctccgcgccggcggctacccctttcctctcgccttctccatcctagctccgcctctcac

SEQ ID NO: 15491 - RNA, 6627 nt, Homo sapiens
  source 1..6627: mol_type = other RNA
gctgggattacaggcatgagccactgtaccaggctgagtccacacttctaagcttgctgttgctctcagacttgcagaacaacctattaaacagaagtaggtaaaagttgagaaagggaagtggccaccacagaaccagttctgctgagaacgaggactcgagtcaggctatgctaccctccttccatggccatgggaaaaaggggtgtgtgctgttggtgtgagagatctggatcttaacagatcagacttaaactaatttgcccatgatgaccgtgtggatttggagggacctgggaatctcacagacctatgggatgtcccagtgatatgtcctgggcttcataccagccctgccctgcctgacaagttggatgaaaactgataaaggacttgtcatagcttcagatggcaaaaccaggccaggccagaatgaaaaaggagaaggaatttaacatgggcaaatgccaagctctgcatttaactaaccaaggctgcttggcgtgaacaaaactgagacagagcaatgcatggagaaaagggttgggcatttgtgggctacaagcttggcatgacatggatgcaaatgtcaatgggtgcacccccagatgcctgtgactccctctggtggtttctgtgcacaacttcccccaaaataggccctacgactccagcagaaacctaccctggggctcctagagcttcctagcctgcctgccagagagcagaagtgcctggaggctacatcttcacccctgggtagtccttactctgaggtgggactgcatccagggctcccctttagggtctgacttggactgaaatcacaccctgccttgccttctgcccctcccttaacttgctctcccctccctaataactccagcatcctcatctcagcagaagcttctggggaacccagcccaagatgagtggtgagggctagggtagccctcctcaatgcactctgggaactacattttcagaagccccagccagagggccaagtcccaggcagggtgcaaagctgtggggcgaggaacctggaaagaggctctgaacaagggacttttaaggaagtgggatgtgggctgtgatcacagccaagctggcagggtaagaggtggcccctgaatgtggctatgagaggggtgcccaacactaccagcctgtgtgctgagcactaactcagtgccaggcactacttgggttattctatttaatctccacaccaagcatgtgaaggaggcaccattgtcatccccatcttacagatgaggaagatgatcaaggcttgtaacttgcccaagatcacatggctataggtgtggatcctatatatccagattcaaactccagctttagcccactaagctacggtggccaaccccagcccaaagtgttgggacctgcgtgtagaagaccccttcagcccttgtaaagttaggatctagcatgtctaaggggacagagacccaatccaggtgacacaggaggtaagatcacagtggaacaggccatccctgcttttccaccaccaccagcactgtgacctcagaccagctctactctatgagtttcttgtgacagtgatggcagcctggggccagacaagggatgcgtgtcttgtgtcctggacacaagacaggcaggcccagaggggacaagctatatgaagagaggcttcagctgtcgggggtcctgaatgccatggaaggagagcaggtgggcagaagcagggagcccctggagcagacagaggggggattcctgctgaggcaaggggctctaggactccagggtttatgctccaaagaacagaatttaccaggacaaaataaacaagaccagtcaggaccgatgccccatccctgctggggtctggcaaagctctcacctccaaatttgtatctgttttgaattcaaagccaaacaaacacatcaacagtgaactccaacacctcccagagcagggcctgaaagggacccagaaagtctggccagaaatctagagtccaaggggaggagatctgtaaactaaaccgctggccatgctctggggccctaaaccactgcaggcatcagggctgttccaggagagggcacagcaaagggggttgggaggggtctccagttccaatcagaaatgaggctgcagtcacttcaggtagacctgtcagcagcagctgtgcaactgggctagggagacaaggatcgtggtttagccaggagaatcatctggggccccagccaagacacaggtgttggatttcagcaccgctctgcaaatactcatctcagtgacgatgaggtgagtgggagcttggctgagcccagcccggcctgccatcctggcaagccagggcagcatggaggtagcacagagtggcacccagccagcgtgaatgcataagaatctgcacgtgacacagaagaaagtctcttcatgaagtaggtttcactggtcccagccaaaccctgtggcaggtggccctttctgcacctgctgaacatgccattcaccttgacccaggtagtggcctcaccctcctcttgctcaaactggaaacctcagcatcctgaaatgcctcctccccaaatccattgcacacatgtgtgcctgtgtatgcgtgtgtgtgcacgtgtatgaacccagcccccagctgcccactccattgcccctaaacaggcccctccttggtgtcacctggcacatctccactggaagccaaatggatatttctaaactgaaatctggtcccacctcagaaccccttccacagttcccttaaagttcctttcctcatttacatcaggatcttcacaatggggacccctggtcacctcccaacccaacaaacgctccaaatgagccgccactgcagaaactcattatggcccaggcaggacaggcacatccaagtatctgaccaggctgttccatctgccaggcaggtcctgccctctctccacccacctgtctaacccctgcatcctcaagaccctacttagctatggccctgtgtgaaaggtccctccccatgcacccacagccatttgttctctctcatgtggccctaacaggctggggttcctggagactccatggggagccaggcatgaagatggcatatacccatgtgtcactccccagaacgtgagctgcctgccctggcaccatacacaaagggactgacagccccagaatcccaaggggtgcacctatgcatatgggaaaggcatgtttacgggtgagaatggtccatcgttgggcttcaggaggcatctgacctgacgcacgcctttgtcactttgtccttgtggcctgttgaaatgccactcctgctttacaaattcaccaactgttgcatgagtcatttccacctcaatgagtaccaggtccttgaggatggggaaaagtaagccaccactgtgggggtcctgggctcctaggtgcagaagaggctccagaaacaggccaggtcgtgggccatgaccccacactagccctctggtccctcacacgggtggattggggggctgtgtcacgggatcttaggatcttcaagacaaagacccaggacaagaacacaagcccactcccattcttcacaggcctcgagaaatctttgggcaatgaagtcagactgtgccaaagcccatgtttctgtctctccaaggcccctggcccccactgcctagcctaggtcaggtcatgtgggcaagcgagcccccacagcctcacagcccctaccccagggccagggcaaactcctgccctgtccccctccattcctgccctccctccttccacaaactgcaccagctggggagaaatccttcagccgacagaatgaggtgaaaatagtgcaattttaggctttgtaactgagattagggcaggtggccacccattctccccttcctcaggccagcctctgacacaatgaccctggaagcctggcagccctccgtaatggtcagcatcctcccctgccatccccaacccacaccatgagctcagccagggcaggggcagcctctgtctcattcaccacagaatccacagaacccagcacagagtatgagctcagtaaattctcctcatacatgactgcactgactggaccgggcacatgctacagggcaacacccacggctcagctggccctggctttggatctcagtcccacctcttcaagctgtccagcgtggggcacatcggctacagccttgccaaatgaaggcttgccaggatgaagaggtgaagacaggacaagcacagtatgtggcacacaggaggcctctgataacatcagtccccttccctaaagacctgggcagtccctgtcactggggcctcacatttcatgtcgagaattcactatttctcagcactgatttcaaataaagccaccaagagtctgacgaggcaacatggcagagttctgagggtggagtgaacaaaaggtcattttttacagaaaactcaggatctcccctctgcacagtgctaaagccctgtctcaaagttcagagcccggaaggtgcagagatgtggcccttggaaatcaagcccttaagaaaacagcccagctgtgtagggccggaagccccaggctgcagtcctgtggtctggaggcagccaatattcaggtgagagatgtgcccagctgccggtgggtccagggggcacggagcccccaccgtccctggcccaggtctaggactaagtcagtgggcccaggccagctccaagggccacagctcctcactcgggggccgcgccggagcagccgcagcagctggggcgccgcagggactgcatgacagcccgcagtggccccctccggccctccacagacaggctgtcctcgctggcgggcgcccgctgcagctgctcaaactgcatctccaggtgcttctggatggccacaccgagcacctccaggtccaccgcagctccgtacacctcccatgtcatgccctcagcatcccatcgcacatcccgcacaggggacggcacctcctccaggctggaccccagagttacctctgggaacacatgcagggctgcaggcgcttccagggacggactggtggccacagccttgcaggccgccactggggccgcctgcacaccagcatcctgggctgacagcggggatgcctctgcaggggccaagtcattggctgaggtcatggtccacacatctttggtcctagagccaggctctgggactaacccagcgggaccccaaaggtgggcacagcaatgggaatgcccagggagccccccagacaacctacagtggatcttcaccccatgctgagcctgcagcccagactcgctcactgacgccactagtttgggaaaggccaggatccctgtggcaggtagggcatggcagcagccaccagccctcacctccctcatgccacagagtagagcagctgggggcagagcatggcaggtggtggtagccagctgttcagcagctttgggctcagcctgggcactgctgctgtgggcagttgtgtcccccaggtctagtggtggcactgacaactgactcgcccccagcatccaggctgagttagaagtctcatcctcaggagccaggtccctttccaggcctgcaggggcctggccaccctggccagaagtaccacctggctgcagctgagccctgtggacagggctgctgccaagggctgagcagctgagactggccttccgagcaccactgtgtccccgcatctgggtgctacggaccaggtctgaatggctcctctgcatagcagcagcactaggggcccgcaggcgacacaggtcactgccgcccatggtggacacattgcccacagtgctgctccaccagtggcctccagcactgggtcgcgccttggggccagaggcccgtgctggcttcatgctctcaggcgggttcccctcttcctccggggcctggggtctggtgctggcctcgcccagctgggcctgccacacggtgctgctggcagtcttgcggagctctggcctctgttcccggccttcacccagcaggctggaagagctctgggacaggggctgaaggcgggggctcaggggtgcccagggacccggctcggggcggctggagctcatggctgcctctagctccaggggcaaggagaggccccatgcatcagctttttccatgagggactcattcagcatctggtcattgattccacagcatctcctgagcccctactgcgtgcccagctgtagggctgatgtgtcgtcggcactcagaggattatctgctgtgtgcctgaccaagagaacaagcaaatacaagaacacacccacagaggagggcactgagtgccaaaaatggggtctgagggagggcaccaccaaggcaggagagctcacggagggtgagagatgagaaaaggcttcctggaggaccagccacgtaagtcaggccttaatgttctctctcctgccccatttgatgccgaagttgctatggttgtggccgatgtcccgtggccaatgccaggctgtcctgctgcctcaggttccacctgtcagcaaccctttcctctcgccttctccatcctagctccgcctctcac

SEQ ID NO: 15492 - RNA, 6548 nt, Homo sapiens
  source 1..6548: mol_type = other RNA
gctgggattacaggcatgagccactgtaccaggctgagtccacacttctaagcttgctgttgctctcagacttgcagaacaacctattaaacagaagtaggtaaaagttgagaaagggaagtggccaccacagaaccagttctgctgagaacgaggactcgagtcaggctatgctaccctccttccatggccatgggaaaaaggggtgtgtgctgttggtgtgagagatctggatcttaacagatcagacttaaactaatttgcccatgatgaccgtgtggatttggagggacctgggaatctcacagacctatgggatgtcccagtgatatgtcctgggcttcataccagccctgccctgcctgacaagttggatgaaaactgataaaggacttgtcatagcttcagatggcaaaaccaggccaggccagaatgaaaaaggagaaggaatttaacatgggcaaatgccaagctctgcatttaactaaccaaggctgcttggcgtgaacaaaactgagacagagcaatgcatggagaaaagggttgggcatttgtgggctacaagcttggcatgacatggatgcaaatgtcaatgggtgcacccccagatgcctgtgactccctctggtggtttctgtgcacaacttcccccaaaataggccctacgactccagcagaaacctaccctggggctcctagagcttcctagcctgcctgccagagagcagaagtgcctggaggctacatcttcacccctgggtagtccttactctgaggtgggactgcatccagggctcccctttagggtctgacttggactgaaatcacaccctgccttgccttctgcccctcccttaacttgctctcccctccctaataactccagcatcctcatctcagcagaagcttctggggaacccagcccaagatgagtggtgagggctagggtagccctcctcaatgcactctgggaactacattttcagaagccccagccagagggccaagtcccaggcagggtgcaaagctgtggggcgaggaacctggaaagaggctctgaacaagggacttttaaggaagtgggatgtgggctgtgatcacagccaagctggcagggtaagaggtggcccctgaatgtggctatgagaggggtgcccaacactaccagcctgtgtgctgagcactaactcagtgccaggcactacttgggttattctatttaatctccacaccaagcatgtgaaggaggcaccattgtcatccccatcttacagatgaggaagatgatcaaggcttgtaacttgcccaagatcacatggctataggtgtggatcctatatatccagattcaaactccagctttagcccactaagctacggtggccaaccccagcccaaagtgttgggacctgcgtgtagaagaccccttcagcccttgtaaagttaggatctagcatgtctaaggggacagagacccaatccaggtgacacaggaggtaagatcacagtggaacaggccatccctgcttttccaccaccaccagcactgtgacctcagaccagctctactctatgagtttcttgtgacagtgatggcagcctggggccagacaagggatgcgtgtcttgtgtcctggacacaagacaggcaggcccagaggggacaagctatatgaagagaggcttcagctgtcgggggtcctgaatgccatggaaggagagcaggtgggcagaagcagggagcccctggagcagacagaggggggattcctgctgaggcaaggggctctaggactccagggtttatgctccaaagaacagaatttaccaggacaaaataaacaagaccagtcaggaccgatgccccatccctgctggggtctggcaaagctctcacctccaaatttgtatctgttttgaattcaaagccaaacaaacacatcaacagtgaactccaacacctcccagagcagggcctgaaagggacccagaaagtctggccagaaatctagagtccaaggggaggagatctgtaaactaaaccgctggccatgctctggggccctaaaccactgcaggcatcagggctgttccaggagagggcacagcaaagggggttgggaggggtctccagttccaatcagaaatgaggctgcagtcacttcaggtagacctgtcagcagcagctgtgcaactgggctagggagacaaggatcgtggtttagccaggagaatcatctggggccccagccaagacacaggtgttggatttcagcaccgctctgcaaatactcatctcagtgacgatgaggtgagtgggagcttggctgagcccagcccggcctgccatcctggcaagccagggcagcatggaggtagcacagagtggcacccagccagcgtgaatgcataagaatctgcacgtgacacagaagaaagtctcttcatgaagtaggtttcactggtcccagccaaaccctgtggcaggtggccctttctgcacctgctgaacatgccattcaccttgacccaggtagtggcctcaccctcctcttgctcaaactggaaacctcagcatcctgaaatgcctcctccccaaatccattgcacacatgtgtgcctgtgtatgcgtgtgtgtgcacgtgtatgaacccagcccccagctgcccactccattgcccctaaacaggcccctccttggtgtcacctggcacatctccactggaagccaaatggatatttctaaactgaaatctggtcccacctcagaaccccttccacagttcccttaaagttcctttcctcatttacatcaggatcttcacaatggggacccctggtcacctcccaacccaacaaacgctccaaatgagccgccactgcagaaactcattatggcccaggcaggacaggcacatccaagtatctgaccaggctgttccatctgccaggcaggtcctgccctctctccacccacctgtctaacccctgcatcctcaagaccctacttagctatggccctgtgtgaaaggtccctccccatgcacccacagccatttgttctctctcatgtggccctaacaggctggggttcctggagactccatggggagccaggcatgaagatggcatatacccatgtgtcactccccagaacgtgagctgcctgccctggcaccatacacaaagggactgacagccccagaatcccaaggggtgcacctatgcatatgggaaaggcatgtttacgggtgagaatggtccatcgttgggcttcaggaggcatctgacctgacgcacgcctttgtcactttgtccttgtggcctgttgaaatgccactcctgctttacaaattcaccaactgttgcatgagtcatttccacctcaatgagtaccaggtccttgaggatggggaaaagtaagccaccactgtgggggtcctgggctcctaggtgcagaagaggctccagaaacaggccaggtcgtgggccatgaccccacactagccctctggtccctcacacgggtggattggggggctgtgtcacgggatcttaggatcttcaagacaaagacccaggacaagaacacaagcccactcccattcttcacaggcctcgagaaatctttgggcaatgaagtcagactgtgccaaagcccatgtttctgtctctccaaggcccctggcccccactgcctagcctaggtcaggtcatgtgggcaagcgagcccccacagcctcacagcccctaccccagggccagggcaaactcctgccctgtccccctccattcctgccctccctccttccacaaactgcaccagctggggagaaatccttcagccgacagaatgaggtgaaaatagtgcaattttaggctttgtaactgagattagggcaggtggccacccattctccccttcctcaggccagcctctgacacaatgaccctggaagcctggcagccctccgtaatggtcagcatcctcccctgccatccccaacccacaccatgagctcagccagggcaggggcagcctctgtctcattcaccacagaatccacagaacccagcacagagtatgagctcagtaaattctcctcatacatgactgcactgactggaccgggcacatgctacagggcaacacccacggctcagctggccctggctttggatctcagtcccacctcttcaagctgtccagcgtggggcacatcggctacagccttgccaaatgaaggcttgccaggatgaagaggtgaagacaggacaagcacagtatgtggcacacaggaggcctctgataacatcagtccccttccctaaagacctgggcagtccctgtcactggggcctcacatttcatgtcgagaattcactatttctcagcactgatttcaaataaagccaccaagagtctgacgaggcaacatggcagagttctgagggtggagtgaacaaaaggtcattttttacagaaaactcaggatctcccctctgcacagtgctaaagccctgtctcaaagttcagagcccggaaggtgcagagatgtggcccttggaaatcaagcccttaagaaaacagcccagctgtgtagggccggaagccccaggctgcagtcctgtggtctggaggcagccaatattcaggtgagagatgtgcccagctgccggtgggtccagggggcacggagcccccaccgtccctggcccaggtctaggactaagtcagtgggcccaggccagctccaagggccacagctcctcactcgggggccgcgccggagcagccgcagcagctggggcgccgcagggactgcatgacagcccgcagtggccccctccggccctccacagacaggctgtcctcgctggcgggcgcccgctgcagctgctcaaactgcatctccaggtgcttctggatggccacaccgagcacctccaggtccaccgcagctccgtacacctcccatgtcatgccctcagcatcccatcgcacatcccgcacaggggacggcacctcctccaggctggaccccagagttacctctgggaacacatgcagggctgcaggcgcttccagggacggactggtggccacagccttgcaggccgccactggggccgcctgcacaccagcatcctgggctgacagcggggatgcctctgcaggggccaagtcattggctgaggtcatggtccacacatctttggtcctagagccaggctctgggactaacccagcgggaccccaaaggtgggcacagcaatgggaatgcccagggagccccccagacaacctacagtggatcttcaccccatgctgagcctgcagcccagactcgctcactgacgccactagtttgggaaaggccaggatccctgtggcaggtagggcatggcagcagccaccagccctcacctccctcatgccacagagtagagcagctgggggcagagcatggcaggtggtggtagccagctgttcagcagctttgggctcagcctgggcactgctgctgtgggcagttgtgtcccccaggtctagtggtggcactgacaactgactcgcccccagcatccaggctgagttagaagtctcatcctcaggagccaggtccctttccaggcctgcaggggcctggccaccctggccagaagtaccacctggctgcagctgagccctgtggacagggctgctgccaagggctgagcagctgagactggccttccgagcaccactgtgtccccgcatctgggtgctacggaccaggtctgaatggctcctctgcatagcagcagcactaggggcccgcaggcgacacaggtcactgccgcccatggtggacacattgcccacagtgctgctccaccagtggcctccagcactgggtcgcgccttggggccagaggcccgtgctggcttcatgctctcaggcgggttcccctcttcctccggggcctggggtctggtgctggcctcgcccagctgggcctgccacacggtgctgctggcagtcttgcggagctctggcctctgttcccggccttcacccagcaggctggaagagctctgggacaggggctgaaggcgggggctcaggggtgcccagggacccggctcggggcggctggagctcatggctgcctctagctccaggggcaaggagaggccccatgcatcagctttttccatgagggactcattcagcatctggtcattgattccacagcatctcctgagcccctactgcgtgcccagctgtagggcttaatgttctctctcctgccccatttgatgccgaagttgctatggttgtggccgatgtcccgtggccaatgccaggctgtcctgctgcctcaggttccacctgtcagcaacctctcgcccgccggggccgcgcaggcgggggaagcgctgctcctgcggccgccacaggtgccaggtgccgcggcccaagatggagccagagccgacctggcctgggcgcgagacgccgcccgccgccgtcggcccggcccgcggagcaagcgccgggtac

SEQ ID NO: 15493 - RNA, 6619 nt, Homo sapiens
  source 1..6619: mol_type = other RNA
gctgggattacaggcatgagccactgtaccaggctgagtccacacttctaagcttgctgttgctctcagacttgcagaacaacctattaaacagaagtaggtaaaagttgagaaagggaagtggccaccacagaaccagttctgctgagaacgaggactcgagtcaggctatgctaccctccttccatggccatgggaaaaaggggtgtgtgctgttggtgtgagagatctggatcttaacagatcagacttaaactaatttgcccatgatgaccgtgtggatttggagggacctgggaatctcacagacctatgggatgtcccagtgatatgtcctgggcttcataccagccctgccctgcctgacaagttggatgaaaactgataaaggacttgtcatagcttcagatggcaaaaccaggccaggccagaatgaaaaaggagaaggaatttaacatgggcaaatgccaagctctgcatttaactaaccaaggctgcttggcgtgaacaaaactgagacagagcaatgcatggagaaaagggttgggcatttgtgggctacaagcttggcatgacatggatgcaaatgtcaatgggtgcacccccagatgcctgtgactccctctggtggtttctgtgcacaacttcccccaaaataggccctacgactccagcagaaacctaccctggggctcctagagcttcctagcctgcctgccagagagcagaagtgcctggaggctacatcttcacccctgggtagtccttactctgaggtgggactgcatccagggctcccctttagggtctgacttggactgaaatcacaccctgccttgccttctgcccctcccttaacttgctctcccctccctaataactccagcatcctcatctcagcagaagcttctggggaacccagcccaagatgagtggtgagggctagggtagccctcctcaatgcactctgggaactacattttcagaagccccagccagagggccaagtcccaggcagggtgcaaagctgtggggcgaggaacctggaaagaggctctgaacaagggacttttaaggaagtgggatgtgggctgtgatcacagccaagctggcagggtaagaggtggcccctgaatgtggctatgagaggggtgcccaacactaccagcctgtgtgctgagcactaactcagtgccaggcactacttgggttattctatttaatctccacaccaagcatgtgaaggaggcaccattgtcatccccatcttacagatgaggaagatgatcaaggcttgtaacttgcccaagatcacatggctataggtgtggatcctatatatccagattcaaactccagctttagcccactaagctacggtggccaaccccagcccaaagtgttgggacctgcgtgtagaagaccccttcagcccttgtaaagttaggatctagcatgtctaaggggacagagacccaatccaggtgacacaggaggtaagatcacagtggaacaggccatccctgcttttccaccaccaccagcactgtgacctcagaccagctctactctatgagtttcttgtgacagtgatggcagcctggggccagacaagggatgcgtgtcttgtgtcctggacacaagacaggcaggcccagaggggacaagctatatgaagagaggcttcagctgtcgggggtcctgaatgccatggaaggagagcaggtgggcagaagcagggagcccctggagcagacagaggggggattcctgctgaggcaaggggctctaggactccagggtttatgctccaaagaacagaatttaccaggacaaaataaacaagaccagtcaggaccgatgccccatccctgctggggtctggcaaagctctcacctccaaatttgtatctgttttgaattcaaagccaaacaaacacatcaacagtgaactccaacacctcccagagcagggcctgaaagggacccagaaagtctggccagaaatctagagtccaaggggaggagatctgtaaactaaaccgctggccatgctctggggccctaaaccactgcaggcatcagggctgttccaggagagggcacagcaaagggggttgggaggggtctccagttccaatcagaaatgaggctgcagtcacttcaggtagacctgtcagcagcagctgtgcaactgggctagggagacaaggatcgtggtttagccaggagaatcatctggggccccagccaagacacaggtgttggatttcagcaccgctctgcaaatactcatctcagtgacgatgaggtgagtgggagcttggctgagcccagcccggcctgccatcctggcaagccagggcagcatggaggtagcacagagtggcacccagccagcgtgaatgcataagaatctgcacgtgacacagaagaaagtctcttcatgaagtaggtttcactggtcccagccaaaccctgtggcaggtggccctttctgcacctgctgaacatgccattcaccttgacccaggtagtggcctcaccctcctcttgctcaaactggaaacctcagcatcctgaaatgcctcctccccaaatccattgcacacatgtgtgcctgtgtatgcgtgtgtgtgcacgtgtatgaacccagcccccagctgcccactccattgcccctaaacaggcccctccttggtgtcacctggcacatctccactggaagccaaatggatatttctaaactgaaatctggtcccacctcagaaccccttccacagttcccttaaagttcctttcctcatttacatcaggatcttcacaatggggacccctggtcacctcccaacccaacaaacgctccaaatgagccgccactgcagaaactcattatggcccaggcaggacaggcacatccaagtatctgaccaggctgttccatctgccaggcaggtcctgccctctctccacccacctgtctaacccctgcatcctcaagaccctacttagctatggccctgtgtgaaaggtccctccccatgcacccacagccatttgttctctctcatgtggccctaacaggctggggttcctggagactccatggggagccaggcatgaagatggcatatacccatgtgtcactccccagaacgtgagctgcctgccctggcaccatacacaaagggactgacagccccagaatcccaaggggtgcacctatgcatatgggaaaggcatgtttacgggtgagaatggtccatcgttgggcttcaggaggcatctgacctgacgcacgcctttgtcactttgtccttgtggcctgttgaaatgccactcctgctttacaaattcaccaactgttgcatgagtcatttccacctcaatgagtaccaggtccttgaggatggggaaaagtaagccaccactgtgggggtcctgggctcctaggtgcagaagaggctccagaaacaggccaggtcgtgggccatgaccccacactagccctctggtccctcacacgggtggattggggggctgtgtcacgggatcttaggatcttcaagacaaagacccaggacaagaacacaagcccactcccattcttcacaggcctcgagaaatctttgggcaatgaagtcagactgtgccaaagcccatgtttctgtctctccaaggcccctggcccccactgcctagcctaggtcaggtcatgtgggcaagcgagcccccacagcctcacagcccctaccccagggccagggcaaactcctgccctgtccccctccattcctgccctccctccttccacaaactgcaccagctggggagaaatccttcagccgacagaatgaggtgaaaatagtgcaattttaggctttgtaactgagattagggcaggtggccacccattctccccttcctcaggccagcctctgacacaatgaccctggaagcctggcagccctccgtaatggtcagcatcctcccctgccatccccaacccacaccatgagctcagccagggcaggggcagcctctgtctcattcaccacagaatccacagaacccagcacagagtatgagctcagtaaattctcctcatacatgactgcactgactggaccgggcacatgctacagggcaacacccacggctcagctggccctggctttggatctcagtcccacctcttcaagctgtccagcgtggggcacatcggctacagccttgccaaatgaaggcttgccaggatgaagaggtgaagacaggacaagcacagtatgtggcacacaggaggcctctgataacatcagtccccttccctaaagacctgggcagtccctgtcactggggcctcacatttcatgtcgagaattcactatttctcagcactgatttcaaataaagccaccaagagtctgacgaggcaacatggcagagttctgagggtggagtgaacaaaaggtcattttttacagaaaactcaggatctcccctctgcacagtgctaaagccctgtctcaaagttcagagcccggaaggtgcagagatgtggcccttggaaatcaagcccttaagaaaacagcccagctgtgtagggccggaagccccaggctgcagtcctgtggtctggaggcagccaatattcaggtgagagatgtgcccagctgccggtgggtccagggggcacggagcccccaccgtccctggcccaggtctaggactaagtcagtgggcccaggccagctccaagggccacagctcctcactcgggggccgcgccggagcagccgcagcagctggggcgccgcagggactgcatgacagcccgcagtggccccctccggccctccacagacaggctgtcctcgctggcgggcgcccgctgcagctgctcaaactgcatctccaggtgcttctggatggccacaccgagcacctccaggtccaccgcagctccgtacacctcccatgtcatgccctcagcatcccatcgcacatcccgcacaggggacggcacctcctccaggctggaccccagagttacctctgggaacacatgcagggctgcaggcgcttccagggacggactggtggccacagccttgcaggccgccactggggccgcctgcacaccagcatcctgggctgacagcggggatgcctctgcaggggccaagtcattggctgaggtcatggtccacacatctttggtcctagagccaggctctgggactaacccagcgggaccccaaaggtgggcacagcaatgggaatgcccagggagccccccagacaacctacagtggatcttcaccccatgctgagcctgcagcccagactcgctcactgacgccactagtttgggaaaggccaggatccctgtggcaggtagggcatggcagcagccaccagccctcacctccctcatgccacagagtagagcagctgggggcagagcatggcaggtggtggtagccagctgttcagcagctttgggctcagcctgggcactgctgctgtgggcagttgtgtcccccaggtctagtggtggcactgacaactgactcgcccccagcatccaggctgagttagaagtctcatcctcaggagccaggtccctttccaggcctgcaggggcctggccaccctggccagaagtaccacctggctgcagctgagccctgtggacagggctgctgccaagggctgagcagctgagactggccttccgagcaccactgtgtccccgcatctgggtgctacggaccaggtctgaatggctcctctgcatagcagcagcactaggggcccgcaggcgacacaggtcactgccgcccatggtggacacattgcccacagtgctgctccaccagtggcctccagcactgggtcgcgccttggggccagaggcccgtgctggcttcatgctctcaggcgggttcccctcttcctccggggcctggggtctggtgctggcctcgcccagctgggcctgccacacggtgctgctggcagtcttgcggagctctggcctctgttcccggccttcacccagcaggctggaagagctctgggacaggggctgaaggcgggggctcaggggtgcccagggacccggctcggggcggctggagctcatggctgcctctagctccaggggcaaggagaggccccatgcatcagctttttccatgagggactcattcagcatctggtcattgattccacagcatctcctgagcccctactgcgtgcccagctgtagggcttaatgttctctctcctgccccatttgatgccgaagttgctatggttgtggccgatgtcccgtggccaatgccaggctgtcctgctgcctcaggttccacctgtcagcaactctcaaggaccaggcaggaatgcacacagcacaaacccccattgcacagtggggatacagcaccctccaggaggtggtttaatccaccccagagtgaacggggcctgataggaacactcagggccaactctgggcaaagcagcaggcagcattccacgccccgcattgaggtctccgcgccggcggctacccctttcctctcgccttctccatcctagctccgcctctcac

SEQ ID NO: 15494 - RNA, 6583 nt, Homo sapiens
  source 1..6583: mol_type = other RNA
gctgggattacaggcatgagccactgtaccaggctgagtccacacttctaagcttgctgttgctctcagacttgcagaacaacctattaaacagaagtaggtaaaagttgagaaagggaagtggccaccacagaaccagttctgctgagaacgaggactcgagtcaggctatgctaccctccttccatggccatgggaaaaaggggtgtgtgctgttggtgtgagagatctggatcttaacagatcagacttaaactaatttgcccatgatgaccgtgtggatttggagggacctgggaatctcacagacctatgggatgtcccagtgatatgtcctgggcttcataccagccctgccctgcctgacaagttggatgaaaactgataaaggacttgtcatagcttcagatggcaaaaccaggccaggccagaatgaaaaaggagaaggaatttaacatgggcaaatgccaagctctgcatttaactaaccaaggctgcttggcgtgaacaaaactgagacagagcaatgcatggagaaaagggttgggcatttgtgggctacaagcttggcatgacatggatgcaaatgtcaatgggtgcacccccagatgcctgtgactccctctggtggtttctgtgcacaacttcccccaaaataggccctacgactccagcagaaacctaccctggggctcctagagcttcctagcctgcctgccagagagcagaagtgcctggaggctacatcttcacccctgggtagtccttactctgaggtgggactgcatccagggctcccctttagggtctgacttggactgaaatcacaccctgccttgccttctgcccctcccttaacttgctctcccctccctaataactccagcatcctcatctcagcagaagcttctggggaacccagcccaagatgagtggtgagggctagggtagccctcctcaatgcactctgggaactacattttcagaagccccagccagagggccaagtcccaggcagggtgcaaagctgtggggcgaggaacctggaaagaggctctgaacaagggacttttaaggaagtgggatgtgggctgtgatcacagccaagctggcagggtaagaggtggcccctgaatgtggctatgagaggggtgcccaacactaccagcctgtgtgctgagcactaactcagtgccaggcactacttgggttattctatttaatctccacaccaagcatgtgaaggaggcaccattgtcatccccatcttacagatgaggaagatgatcaaggcttgtaacttgcccaagatcacatggctataggtgtggatcctatatatccagattcaaactccagctttagcccactaagctacggtggccaaccccagcccaaagtgttgggacctgcgtgtagaagaccccttcagcccttgtaaagttaggatctagcatgtctaaggggacagagacccaatccaggtgacacaggaggtaagatcacagtggaacaggccatccctgcttttccaccaccaccagcactgtgacctcagaccagctctactctatgagtttcttgtgacagtgatggcagcctggggccagacaagggatgcgtgtcttgtgtcctggacacaagacaggcaggcccagaggggacaagctatatgaagagaggcttcagctgtcgggggtcctgaatgccatggaaggagagcaggtgggcagaagcagggagcccctggagcagacagaggggggattcctgctgaggcaaggggctctaggactccagggtttatgctccaaagaacagaatttaccaggacaaaataaacaagaccagtcaggaccgatgccccatccctgctggggtctggcaaagctctcacctccaaatttgtatctgttttgaattcaaagccaaacaaacacatcaacagtgaactccaacacctcccagagcagggcctgaaagggacccagaaagtctggccagaaatctagagtccaaggggaggagatctgtaaactaaaccgctggccatgctctggggccctaaaccactgcaggcatcagggctgttccaggagagggcacagcaaagggggttgggaggggtctccagttccaatcagaaatgaggctgcagtcacttcaggtagacctgtcagcagcagctgtgcaactgggctagggagacaaggatcgtggtttagccaggagaatcatctggggccccagccaagacacaggtgttggatttcagcaccgctctgcaaatactcatctcagtgacgatgaggtgagtgggagcttggctgagcccagcccggcctgccatcctggcaagccagggcagcatggaggtagcacagagtggcacccagccagcgtgaatgcataagaatctgcacgtgacacagaagaaagtctcttcatgaagtaggtttcactggtcccagccaaaccctgtggcaggtggccctttctgcacctgctgaacatgccattcaccttgacccaggtagtggcctcaccctcctcttgctcaaactggaaacctcagcatcctgaaatgcctcctccccaaatccattgcacacatgtgtgcctgtgtatgcgtgtgtgtgcacgtgtatgaacccagcccccagctgcccactccattgcccctaaacaggcccctccttggtgtcacctggcacatctccactggaagccaaatggatatttctaaactgaaatctggtcccacctcagaaccccttccacagttcccttaaagttcctttcctcatttacatcaggatcttcacaatggggacccctggtcacctcccaacccaacaaacgctccaaatgagccgccactgcagaaactcattatggcccaggcaggacaggcacatccaagtatctgaccaggctgttccatctgccaggcaggtcctgccctctctccacccacctgtctaacccctgcatcctcaagaccctacttagctatggccctgtgtgaaaggtccctccccatgcacccacagccatttgttctctctcatgtggccctaacaggctggggttcctggagactccatggggagccaggcatgaagatggcatatacccatgtgtcactccccagaacgtgagctgcctgccctggcaccatacacaaagggactgacagccccagaatcccaaggggtgcacctatgcatatgggaaaggcatgtttacgggtgagaatggtccatcgttgggcttcaggaggcatctgacctgacgcacgcctttgtcactttgtccttgtggcctgttgaaatgccactcctgctttacaaattcaccaactgttgcatgagtcatttccacctcaatgagtaccaggtccttgaggatggggaaaagtaagccaccactgtgggggtcctgggctcctaggtgcagaagaggctccagaaacaggccaggtcgtgggccatgaccccacactagccctctggtccctcacacgggtggattggggggctgtgtcacgggatcttaggatcttcaagacaaagacccaggacaagaacacaagcccactcccattcttcacaggcctcgagaaatctttgggcaatgaagtcagactgtgccaaagcccatgtttctgtctctccaaggcccctggcccccactgcctagcctaggtcaggtcatgtgggcaagcgagcccccacagcctcacagcccctaccccagggccagggcaaactcctgccctgtccccctccattcctgccctccctccttccacaaactgcaccagctggggagaaatccttcagccgacagaatgaggtgaaaatagtgcaattttaggctttgtaactgagattagggcaggtggccacccattctccccttcctcaggccagcctctgacacaatgaccctggaagcctggcagccctccgtaatggtcagcatcctcccctgccatccccaacccacaccatgagctcagccagggcaggggcagcctctgtctcattcaccacagaatccacagaacccagcacagagtatgagctcagtaaattctcctcatacatgactgcactgactggaccgggcacatgctacagggcaacacccacggctcagctggccctggctttggatctcagtcccacctcttcaagctgtccagcgtggggcacatcggctacagccttgccaaatgaaggcttgccaggatgaagaggtgaagacaggacaagcacagtatgtggcacacaggaggcctctgataacatcagtccccttccctaaagacctgggcagtccctgtcactggggcctcacatttcatgtcgagaattcactatttctcagcactgatttcaaataaagccaccaagagtctgacgaggcaacatggcagagttctgagggtggagtgaacaaaaggtcattttttacagaaaactcaggatctcccctctgcacagtgctaaagccctgtctcaaagttcagagcccggaaggtgcagagatgtggcccttggaaatcaagcccttaagaaaacagcccagctgtgtagggccggaagccccaggctgcagtcctgtggtctggaggcagccaatattcaggtgagagatgtgcccagctgccggtgggtccagggggcacggagcccccaccgtccctggcccaggtctaggactaagtcagtgggcccaggccagctccaagggccacagctcctcactcgggggccgcgccggagcagccgcagcagctggggcgccgcagggactgcatgacagcccgcagtggccccctccggccctccacagacaggctgtcctcgctggcgggcgcccgctgcagctgctcaaactgcatctccaggtgcttctggatggccacaccgagcacctccaggtccaccgcagctccgtacacctcccatgtcatgccctcagcatcccatcgcacatcccgcacaggggacggcacctcctccaggctggaccccagagttacctctgggaacacatgcagggctgcaggcgcttccagggacggactggtggccacagccttgcaggccgccactggggccgcctgcacaccagcatcctgggctgacagcggggatgcctctgcaggggccaagtcattggctgaggtcatggtccacacatctttggtcctagagccaggctctgggactaacccagcgggaccccaaaggtgggcacagcaatgggaatgcccagggagccccccagacaacctacagtggatcttcaccccatgctgagcctgcagcccagactcgctcactgacgccactagtttgggaaaggccaggatccctgtggcaggtagggcatggcagcagccaccagccctcacctccctcatgccacagagtagagcagctgggggcagagcatggcaggtggtggtagccagctgttcagcagctttgggctcagcctgggcactgctgctgtgggcagttgtgtcccccaggtctagtggtggcactgacaactgactcgcccccagcatccaggctgagttagaagtctcatcctcaggagccaggtccctttccaggcctgcaggggcctggccaccctggccagaagtaccacctggctgcagctgagccctgtggacagggctgctgccaagggctgagcagctgagactggccttccgagcaccactgtgtccccgcatctgggtgctacggaccaggtctgaatggctcctctgcatagcagcagcactaggggcccgcaggcgacacaggtcactgccgcccatggtggacacattgcccacagtgctgctccaccagtggcctccagcactgggtcgcgccttggggccagaggcccgtgctggcttcatgctctcaggcgggttcccctcttcctccggggcctggggtctggtgctggcctcgcccagctgggcctgccacacggtgctgctggcagtcttgcggagctctggcctctgttcccggccttcacccagcaggctggaagagctctgggacaggggctgaaggcgggggctcaggggtgcccagggacccggctcggggcggctggagctcatggctgcctctagctccaggggcaaggagaggccccatgcatcagctttttccatgagggactcattcagcatctggtcattgattccacagcatctcctgagcccctactgcgtgcccagctgtagggcttaatgttctctctcctgccccatttgatgccgaagttgctatggttgtggccgatgtcccgtggccaatgccaggctgtcctgctgcctcaggttccacctgtcagcaactctcaaggaccaggcaggaatgcacacagcacaaacccccattgcacagtggggatacagcaccctccaggaggtggtttaatccaccccagagtgaacggggcctgataggaacactcagggccaactctgggcaaagcagcaggcagcattcccctttcctctcgccttctccatcctagctccgcctctcac

SEQ ID NO: 15495 - RNA, 6703 nt, Homo sapiens
  source 1..6703: mol_type = other RNA
gctgggattacaggcatgagccactgtaccaggctgagtccacacttctaagcttgctgttgctctcagacttgcagaacaacctattaaacagaagtaggtaaaagttgagaaagggaagtggccaccacagaaccagttctgctgagaacgaggactcgagtcaggctatgctaccctccttccatggccatgggaaaaaggggtgtgtgctgttggtgtgagagatctggatcttaacagatcagacttaaactaatttgcccatgatgaccgtgtggatttggagggacctgggaatctcacagacctatgggatgtcccagtgatatgtcctgggcttcataccagccctgccctgcctgacaagttggatgaaaactgataaaggacttgtcatagcttcagatggcaaaaccaggccaggccagaatgaaaaaggagaaggaatttaacatgggcaaatgccaagctctgcatttaactaaccaaggctgcttggcgtgaacaaaactgagacagagcaatgcatggagaaaagggttgggcatttgtgggctacaagcttggcatgacatggatgcaaatgtcaatgggtgcacccccagatgcctgtgactccctctggtggtttctgtgcacaacttcccccaaaataggccctacgactccagcagaaacctaccctggggctcctagagcttcctagcctgcctgccagagagcagaagtgcctggaggctacatcttcacccctgggtagtccttactctgaggtgggactgcatccagggctcccctttagggtctgacttggactgaaatcacaccctgccttgccttctgcccctcccttaacttgctctcccctccctaataactccagcatcctcatctcagcagaagcttctggggaacccagcccaagatgagtggtgagggctagggtagccctcctcaatgcactctgggaactacattttcagaagccccagccagagggccaagtcccaggcagggtgcaaagctgtggggcgaggaacctggaaagaggctctgaacaagggacttttaaggaagtgggatgtgggctgtgatcacagccaagctggcagggtaagaggtggcccctgaatgtggctatgagaggggtgcccaacactaccagcctgtgtgctgagcactaactcagtgccaggcactacttgggttattctatttaatctccacaccaagcatgtgaaggaggcaccattgtcatccccatcttacagatgaggaagatgatcaaggcttgtaacttgcccaagatcacatggctataggtgtggatcctatatatccagattcaaactccagctttagcccactaagctacggtggccaaccccagcccaaagtgttgggacctgcgtgtagaagaccccttcagcccttgtaaagttaggatctagcatgtctaaggggacagagacccaatccaggtgacacaggaggtaagatcacagtggaacaggccatccctgcttttccaccaccaccagcactgtgacctcagaccagctctactctatgagtttcttgtgacagtgatggcagcctggggccagacaagggatgcgtgtcttgtgtcctggacacaagacaggcaggcccagaggggacaagctatatgaagagaggcttcagctgtcgggggtcctgaatgccatggaaggagagcaggtgggcagaagcagggagcccctggagcagacagaggggggattcctgctgaggcaaggggctctaggactccagggtttatgctccaaagaacagaatttaccaggacaaaataaacaagaccagtcaggaccgatgccccatccctgctggggtctggcaaagctctcacctccaaatttgtatctgttttgaattcaaagccaaacaaacacatcaacagtgaactccaacacctcccagagcagggcctgaaagggacccagaaagtctggccagaaatctagagtccaaggggaggagatctgtaaactaaaccgctggccatgctctggggccctaaaccactgcaggcatcagggctgttccaggagagggcacagcaaagggggttgggaggggtctccagttccaatcagaaatgaggctgcagtcacttcaggtagacctgtcagcagcagctgtgcaactgggctagggagacaaggatcgtggtttagccaggagaatcatctggggccccagccaagacacaggtgttggatttcagcaccgctctgcaaatactcatctcagtgacgatgaggtgagtgggagcttggctgagcccagcccggcctgccatcctggcaagccagggcagcatggaggtagcacagagtggcacccagccagcgtgaatgcataagaatctgcacgtgacacagaagaaagtctcttcatgaagtaggtttcactggtcccagccaaaccctgtggcaggtggccctttctgcacctgctgaacatgccattcaccttgacccaggtagtggcctcaccctcctcttgctcaaactggaaacctcagcatcctgaaatgcctcctccccaaatccattgcacacatgtgtgcctgtgtatgcgtgtgtgtgcacgtgtatgaacccagcccccagctgcccactccattgcccctaaacaggcccctccttggtgtcacctggcacatctccactggaagccaaatggatatttctaaactgaaatctggtcccacctcagaaccccttccacagttcccttaaagttcctttcctcatttacatcaggatcttcacaatggggacccctggtcacctcccaacccaacaaacgctccaaatgagccgccactgcagaaactcattatggcccaggcaggacaggcacatccaagtatctgaccaggctgttccatctgccaggcaggtcctgccctctctccacccacctgtctaacccctgcatcctcaagaccctacttagctatggccctgtgtgaaaggtccctccccatgcacccacagccatttgttctctctcatgtggccctaacaggctggggttcctggagactccatggggagccaggcatgaagatggcatatacccatgtgtcactccccagaacgtgagctgcctgccctggcaccatacacaaagggactgacagccccagaatcccaaggggtgcacctatgcatatgggaaaggcatgtttacgggtgagaatggtccatcgttgggcttcaggaggcatctgacctgacgcacgcctttgtcactttgtccttgtggcctgttgaaatgccactcctgctttacaaattcaccaactgttgcatgagtcatttccacctcaatgagtaccaggtccttgaggatggggaaaagtaagccaccactgtgggggtcctgggctcctaggtgcagaagaggctccagaaacaggccaggtcgtgggccatgaccccacactagccctctggtccctcacacgggtggattggggggctgtgtcacgggatcttaggatcttcaagacaaagacccaggacaagaacacaagcccactcccattcttcacaggcctcgagaaatctttgggcaatgaagtcagactgtgccaaagcccatgtttctgtctctccaaggcccctggcccccactgcctagcctaggtcaggtcatgtgggcaagcgagcccccacagcctcacagcccctaccccagggccagggcaaactcctgccctgtccccctccattcctgccctccctccttccacaaactgcaccagctggggagaaatccttcagccgacagaatgaggtgaaaatagtgcaattttaggctttgtaactgagattagggcaggtggccacccattctccccttcctcaggccagcctctgacacaatgaccctggaagcctggcagccctccgtaatggtcagcatcctcccctgccatccccaacccacaccatgagctcagccagggcaggggcagcctctgtctcattcaccacagaatccacagaacccagcacagagtatgagctcagtaaattctcctcatacatgactgcactgactggaccgggcacatgctacagggcaacacccacggctcagctggccctggctttggatctcagtcccacctcttcaagctgtccagcgtggggcacatcggctacagccttgccaaatgaaggcttgccaggatgaagaggtgaagacaggacaagcacagtatgtggcacacaggaggcctctgataacatcagtccccttccctaaagacctgggcagtccctgtcactggggcctcacatttcatgtcgagaattcactatttctcagcactgatttcaaataaagccaccaagagtctgacgaggcaacatggcagagttctgagggtggagtgaacaaaaggtcattttttacagaaaactcaggatctcccctctgcacagtgctaaagccctgtctcaaagttcagagcccggaaggtgcagagatgtggcccttggaaatcaagcccttaagaaaacagcccagctgtgtagggccggaagccccaggctgcagtcctgtggtctggaggcagccaatattcaggtgagagatgtgcccagctgccggtgggtccagggggcacggagcccccaccgtccctggcccaggtctaggactaagtcagtgggcccaggccagctccaagggccacagctcctcactcgggggccgcgccggagcagccgcagcagctggggcgccgcagggactgcatgacagcccgcagtggccccctccggccctccacagacaggctgtcctcgctggcgggcgcccgctgcagctgctcaaactgcatctccaggtgcttctggatggccacaccgagcacctccaggtccaccgcagctccgtacacctcccatgtcatgccctcagcatcccatcgcacatcccgcacaggggacggcacctcctccaggctggaccccagagttacctctgggaacacatgcagggctgcaggcgcttccagggacggactggtggccacagccttgcaggccgccactggggccgcctgcacaccagcatcctgggctgacagcggggatgcctctgcaggggccaagtcattggctgaggtcatggtccacacatctttggtcctagagccaggctctgggactaacccagcgggaccccaaaggtgggcacagcaatgggaatgcccagggagccccccagacaacctacagtggatcttcaccccatgctgagcctgcagcccagactcgctcactgacgccactagtttgggaaaggccaggatccctgtggcaggtagggcatggcagcagccaccagccctcacctccctcatgccacagagtagagcagctgggggcagagcatggcaggtggtggtagccagctgttcagcagctttgggctcagcctgggcactgctgctgtgggcagttgtgtcccccaggtctagtggtggcactgacaactgactcgcccccagcatccaggctgagttagaagtctcatcctcaggagccaggtccctttccaggcctgcaggggcctggccaccctggccagaagtaccacctggctgcagctgagccctgtggacagggctgctgccaagggctgagcagctgagactggccttccgagcaccactgtgtccccgcatctgggtgctacggaccaggtctgaatggctcctctgcatagcagcagcactaggggcccgcaggcgacacaggtcactgccgcccatggtggacacattgcccacagtgctgctccaccagtggcctccagcactgggtcgcgccttggggccagaggcccgtgctggcttcatgctctcaggcgggttcccctcttcctccggggcctggggtctggtgctggcctcgcccagctgggcctgccacacggtgctgctggcagtcttgcggagctctggcctctgttcccggccttcacccagcaggctggaagagctctgggacaggggctgaaggcgggggctcaggggtgcccagggacccggctcggggcggctggagctcatggctgcctctagctccaggggcaaggagaggccccatgcatcagctttttccatgagggactcattcagcatctggtcattgattccacagcatctcctgagcccctactgcgtgcccagctgtagggcttaatgttctctctcctgccccatttgatgccgaagttgctatggttgtggccgatgtcccgtggccaatgccaggctgtcctgctgcctcaggttccacctgtcagcaactctcaaggaccaggcaggaatgcacacagcacaaacccccattgcacagtggggatacagcaccctccaggaggtggtttaatccaccccagagtgaacggggcctgataggaacactcagggccaactctgggcaaagcagcaggcagcattccctctcgcccgccggggccgcgcaggcgggggaagcgctgctcctgcggccgccacaggtgccaggtgccgcggcccaagatggagccagagccgacctggcctgggcgcgagacgccgcccgccgccgtcggcccggcccgcggagcaagcgccgggtac

SEQ ID NO: 15496 - RNA, 7054 nt, Homo sapiens
  source 1..7054: mol_type = other RNA
gctgggattacaggcatgagccactgtaccaggctgagtccacacttctaagcttgctgttgctctcagacttgcagaacaacctattaaacagaagtaggtaaaagttgagaaagggaagtggccaccacagaaccagttctgctgagaacgaggactcgagtcaggctatgctaccctccttccatggccatgggaaaaaggggtgtgtgctgttggtgtgagagatctggatcttaacagatcagacttaaactaatttgcccatgatgaccgtgtggatttggagggacctgggaatctcacagacctatgggatgtcccagtgatatgtcctgggcttcataccagccctgccctgcctgacaagttggatgaaaactgataaaggacttgtcatagcttcagatggcaaaaccaggccaggccagaatgaaaaaggagaaggaatttaacatgggcaaatgccaagctctgcatttaactaaccaaggctgcttggcgtgaacaaaactgagacagagcaatgcatggagaaaagggttgggcatttgtgggctacaagcttggcatgacatggatgcaaatgtcaatgggtgcacccccagatgcctgtgactccctctggtggtttctgtgcacaacttcccccaaaataggccctacgactccagcagaaacctaccctggggctcctagagcttcctagcctgcctgccagagagcagaagtgcctggaggctacatcttcacccctgggtagtccttactctgaggtgggactgcatccagggctcccctttagggtctgacttggactgaaatcacaccctgccttgccttctgcccctcccttaacttgctctcccctccctaataactccagcatcctcatctcagcagaagcttctggggaacccagcccaagatgagtggtgagggctagggtagccctcctcaatgcactctgggaactacattttcagaagccccagccagagggccaagtcccaggcagggtgcaaagctgtggggcgaggaacctggaaagaggctctgaacaagggacttttaaggaagtgggatgtgggctgtgatcacagccaagctggcagggtaagaggtggcccctgaatgtggctatgagaggggtgcccaacactaccagcctgtgtgctgagcactaactcagtgccaggcactacttgggttattctatttaatctccacaccaagcatgtgaaggaggcaccattgtcatccccatcttacagatgaggaagatgatcaaggcttgtaacttgcccaagatcacatggctataggtgtggatcctatatatccagattcaaactccagctttagcccactaagctacggtggccaaccccagcccaaagtgttgggacctgcgtgtagaagaccccttcagcccttgtaaagttaggatctagcatgtctaaggggacagagacccaatccaggtgacacaggaggtaagatcacagtggaacaggccatccctgcttttccaccaccaccagcactgtgacctcagaccagctctactctatgagtttcttgtgacagtgatggcagcctggggccagacaagggatgcgtgtcttgtgtcctggacacaagacaggcaggcccagaggggacaagctatatgaagagaggcttcagctgtcgggggtcctgaatgccatggaaggagagcaggtgggcagaagcagggagcccctggagcagacagaggggggattcctgctgaggcaaggggctctaggactccagggtttatgctccaaagaacagaatttaccaggacaaaataaacaagaccagtcaggaccgatgccccatccctgctggggtctggcaaagctctcacctccaaatttgtatctgttttgaattcaaagccaaacaaacacatcaacagtgaactccaacacctcccagagcagggcctgaaagggacccagaaagtctggccagaaatctagagtccaaggggaggagatctgtaaactaaaccgctggccatgctctggggccctaaaccactgcaggcatcagggctgttccaggagagggcacagcaaagggggttgggaggggtctccagttccaatcagaaatgaggctgcagtcacttcaggtagacctgtcagcagcagctgtgcaactgggctagggagacaaggatcgtggtttagccaggagaatcatctggggccccagccaagacacaggtgttggatttcagcaccgctctgcaaatactcatctcagtgacgatgaggtgagtgggagcttggctgagcccagcccggcctgccatcctggcaagccagggcagcatggaggtagcacagagtggcacccagccagcgtgaatgcataagaatctgcacgtgacacagaagaaagtctcttcatgaagtaggtttcactggtcccagccaaaccctgtggcaggtggccctttctgcacctgctgaacatgccattcaccttgacccaggtagtggcctcaccctcctcttgctcaaactggaaacctcagcatcctgaaatgcctcctccccaaatccattgcacacatgtgtgcctgtgtatgcgtgtgtgtgcacgtgtatgaacccagcccccagctgcccactccattgcccctaaacaggcccctccttggtgtcacctggcacatctccactggaagccaaatggatatttctaaactgaaatctggtcccacctcagaaccccttccacagttcccttaaagttcctttcctcatttacatcaggatcttcacaatggggacccctggtcacctcccaacccaacaaacgctccaaatgagccgccactgcagaaactcattatggcccaggcaggacaggcacatccaagtatctgaccaggctgttccatctgccaggcaggtcctgccctctctccacccacctgtctaacccctgcatcctcaagaccctacttagctatggccctgtgtgaaaggtccctccccatgcacccacagccatttgttctctctcatgtggccctaacaggctggggttcctggagactccatggggagccaggcatgaagatggcatatacccatgtgtcactccccagaacgtgagctgcctgccctggcaccatacacaaagggactgacagccccagaatcccaaggggtgcacctatgcatatgggaaaggcatgtttacgggtgagaatggtccatcgttgggcttcaggaggcatctgacctgacgcacgcctttgtcactttgtccttgtggcctgttgaaatgccactcctgctttacaaattcaccaactgttgcatgagtcatttccacctcaatgagtaccaggtccttgaggatggggaaaagtaagccaccactgtgggggtcctgggctcctaggtgcagaagaggctccagaaacaggccaggtcgtgggccatgaccccacactagccctctggtccctcacacgggtggattggggggctgtgtcacgggatcttaggatcttcaagacaaagacccaggacaagaacacaagcccactcccattcttcacaggcctcgagaaatctttgggcaatgaagtcagactgtgccaaagcccatgtttctgtctctccaaggcccctggcccccactgcctagcctaggtcaggtcatgtgggcaagcgagcccccacagcctcacagcccctaccccagggccagggcaaactcctgccctgtccccctccattcctgccctccctccttccacaaactgcaccagctggggagaaatccttcagccgacagaatgaggtgaaaatagtgcaattttaggctttgtaactgagattagggcaggtggccacccattctccccttcctcaggccagcctctgacacaatgaccctggaagcctggcagccctccgtaatggtcagcatcctcccctgccatccccaacccacaccatgagctcagccagggcaggggcagcctctgtctcattcaccacagaatccacagaacccagcacagagtatgagctcagtaaattctcctcatacatgactgcactgactggaccgggcacatgctacagggcaacacccacggctcagctggccctggctttggatctcagtcccacctcttcaagctgtccagcgtggggcacatcggctacagccttgccaaatgaaggcttgccaggatgaagaggtgaagacaggacaagcacagtatgtggcacacaggaggcctctgataacatcagtccccttccctaaagacctgggcagtccctgtcactggggcctcacatttcatgtcgagaattcactatttctcagcactgatttcaaataaagccaccaagagtctgacgaggcaacatggcagagttctgagggtggagtgaacaaaaggtcattttttacagaaaactcaggatctcccctctgcacagtgctaaagccctgtctcaaagttcagagcccggaaggtgcagagatgtggcccttggaaatcaagcccttaagaaaacagcccagctgtgtagggccggaagccccaggctgcagtcctgtggtctggaggcagccaatattcaggtgagagatgtgcccagctgccggtgggtccagggggcacggagcccccaccgtccctggcccaggtctaggactaagtcagtgggcccaggccagctccaagggccacagctcctcactcgggggccgcgccggagcagccgcagcagctggggcgccgcagggactgcatgacagcccgcagtggccccctccggccctccacagacaggctgtcctcgctggcgggcgcccgctgcagctgctcaaactgcatctccaggtgcttctggatggccacaccgagcacctccaggtccaccgcagctccgtacacctcccatgtcatgccctcagcatcccatcgcacatcccgcacaggggacggcacctcctccaggctggaccccagagttacctctgggaacacatgcagggctgcaggcgcttccagggacggactggtggccacagccttgcaggccgccactggggccgcctgcacaccagcatcctgggctgacagcggggatgcctctgcaggggccaagtcattggctgaggtcatggtccacacatctttggtcctagagccaggctctgggactaacccagcgggaccccaaaggtgggcacagcaatgggaatgcccagggagccccccagacaacctacagtggatcttcaccccatgctgagcctgcagcccagactcgctcactgacgccactagtttgggaaaggccaggatccctgtggcaggtagggcatggcagcagccaccagccctcacctccctcatgccacagagtagagcagctgggggcagagcatggcaggtggtggtagccagctgttcagcagctttgggctcagcctgggcactgctgctgtgggcagttgtgtcccccaggtctagtggtggcactgacaactgactcgcccccagcatccaggctgagttagaagtctcatcctcaggagccaggtccctttccaggcctgcaggggcctggccaccctggccagaagtaccacctggctgcagctgagccctgtggacagggctgctgccaagggctgagcagctgagactggccttccgagcaccactgtgtccccgcatctgggtgctacggaccaggtctgaatggctcctctgcatagcagcagcactaggggcccgcaggcgacacaggtcactgccgcccatggtggacacattgcccacagtgctgctccaccagtggcctccagcactgggtcgcgccttggggccagaggcccgtgctggcttcatgctctcaggcgggttcccctcttcctccggggcctggggtctggtgctggcctcgcccagctgggcctgccacacggtgctgctggcagtcttgcggagctctggcctctgttcccggccttcacccagcaggctggaagagctctgggacaggggctgaaggcgggggctcaggggtgcccagggacccggctcggggcggctggagctcatggctgcctctagctccaggggcaaggagaggccccatgcatcagctttttccatgagggactcattcagcatctggtcattgattccacagcatctcctgagcccctactgcgtgcccagctgtagggcttaatgttctctctcctgccccatttgatgccgaagttgctatggttgtggccgatgtcccgtggccaatgccaggctgtcctgctgcctcaggttccacctgtcagcaactctcaaggaccaggcaggaatgcacacagcacaaacccccattgcacagtggggatacagcaccctccaggaggtggtttaatccaccccagagtgaacggggcctgataggaacactcagggccaactctgggcaaagcagcaggcagcattcctaaagggagggtttggaggagacaaaacctgcccttcacaatgaacgtgccttaagggctacatgccccgggtcacaagctgtgccaggaaagggttctggggtaactgtggggtcagtggccccatggatgaggctctgctcaccaggaagaggcctaggcgcccaacagcccctgagcttcctcccctggggaggatttgcccacaatccctggggggcacctaggtggagagggtgccccggcctagaagcagcctaggcggccggtgtgtccctatctgcacgctcacaagcactcatgccccagcctgggacacacaggcccgtatgcagtaacagcgtctacccagctgcactctgcacgccaagcacaggccgcccctgctgcggggccaaaggcctgaaagcaccgcaccacgcagcctcgcccagaatagctcccctcccgcccctcctgcacaaagcccacccggacttagggagaagggggctcaatacgggcccgaaac

SEQ ID NO: 15497 - RNA, 6635 nt, Homo sapiens
  source 1..6635: mol_type = other RNA
gctgggattacaggcatgagccactgtaccaggctgagtccacacttctaagcttgctgttgctctcagacttgcagaacaacctattaaacagaagtaggtaaaagttgagaaagggaagtggccaccacagaaccagttctgctgagaacgaggactcgagtcaggctatgctaccctccttccatggccatgggaaaaaggggtgtgtgctgttggtgtgagagatctggatcttaacagatcagacttaaactaatttgcccatgatgaccgtgtggatttggagggacctgggaatctcacagacctatgggatgtcccagtgatatgtcctgggcttcataccagccctgccctgcctgacaagttggatgaaaactgataaaggacttgtcatagcttcagatggcaaaaccaggccaggccagaatgaaaaaggagaaggaatttaacatgggcaaatgccaagctctgcatttaactaaccaaggctgcttggcgtgaacaaaactgagacagagcaatgcatggagaaaagggttgggcatttgtgggctacaagcttggcatgacatggatgcaaatgtcaatgggtgcacccccagatgcctgtgactccctctggtggtttctgtgcacaacttcccccaaaataggccctacgactccagcagaaacctaccctggggctcctagagcttcctagcctgcctgccagagagcagaagtgcctggaggctacatcttcacccctgggtagtccttactctgaggtgggactgcatccagggctcccctttagggtctgacttggactgaaatcacaccctgccttgccttctgcccctcccttaacttgctctcccctccctaataactccagcatcctcatctcagcagaagcttctggggaacccagcccaagatgagtggtgagggctagggtagccctcctcaatgcactctgggaactacattttcagaagccccagccagagggccaagtcccaggcagggtgcaaagctgtggggcgaggaacctggaaagaggctctgaacaagggacttttaaggaagtgggatgtgggctgtgatcacagccaagctggcagggtaagaggtggcccctgaatgtggctatgagaggggtgcccaacactaccagcctgtgtgctgagcactaactcagtgccaggcactacttgggttattctatttaatctccacaccaagcatgtgaaggaggcaccattgtcatccccatcttacagatgaggaagatgatcaaggcttgtaacttgcccaagatcacatggctataggtgtggatcctatatatccagattcaaactccagctttagcccactaagctacggtggccaaccccagcccaaagtgttgggacctgcgtgtagaagaccccttcagcccttgtaaagttaggatctagcatgtctaaggggacagagacccaatccaggtgacacaggaggtaagatcacagtggaacaggccatccctgcttttccaccaccaccagcactgtgacctcagaccagctctactctatgagtttcttgtgacagtgatggcagcctggggccagacaagggatgcgtgtcttgtgtcctggacacaagacaggcaggcccagaggggacaagctatatgaagagaggcttcagctgtcgggggtcctgaatgccatggaaggagagcaggtgggcagaagcagggagcccctggagcagacagaggggggattcctgctgaggcaaggggctctaggactccagggtttatgctccaaagaacagaatttaccaggacaaaataaacaagaccagtcaggaccgatgccccatccctgctggggtctggcaaagctctcacctccaaatttgtatctgttttgaattcaaagccaaacaaacacatcaacagtgaactccaacacctcccagagcagggcctgaaagggacccagaaagtctggccagaaatctagagtccaaggggaggagatctgtaaactaaaccgctggccatgctctggggccctaaaccactgcaggcatcagggctgttccaggagagggcacagcaaagggggttgggaggggtctccagttccaatcagaaatgaggctgcagtcacttcaggtagacctgtcagcagcagctgtgcaactgggctagggagacaaggatcgtggtttagccaggagaatcatctggggccccagccaagacacaggtgttggatttcagcaccgctctgcaaatactcatctcagtgacgatgaggtgagtgggagcttggctgagcccagcccggcctgccatcctggcaagccagggcagcatggaggtagcacagagtggcacccagccagcgtgaatgcataagaatctgcacgtgacacagaagaaagtctcttcatgaagtaggtttcactggtcccagccaaaccctgtggcaggtggccctttctgcacctgctgaacatgccattcaccttgacccaggtagtggcctcaccctcctcttgctcaaactggaaacctcagcatcctgaaatgcctcctccccaaatccattgcacacatgtgtgcctgtgtatgcgtgtgtgtgcacgtgtatgaacccagcccccagctgcccactccattgcccctaaacaggcccctccttggtgtcacctggcacatctccactggaagccaaatggatatttctaaactgaaatctggtcccacctcagaaccccttccacagttcccttaaagttcctttcctcatttacatcaggatcttcacaatggggacccctggtcacctcccaacccaacaaacgctccaaatgagccgccactgcagaaactcattatggcccaggcaggacaggcacatccaagtatctgaccaggctgttccatctgccaggcaggtcctgccctctctccacccacctgtctaacccctgcatcctcaagaccctacttagctatggccctgtgtgaaaggtccctccccatgcacccacagccatttgttctctctcatgtggccctaacaggctggggttcctggagactccatggggagccaggcatgaagatggcatatacccatgtgtcactccccagaacgtgagctgcctgccctggcaccatacacaaagggactgacagccccagaatcccaaggggtgcacctatgcatatgggaaaggcatgtttacgggtgagaatggtccatcgttgggcttcaggaggcatctgacctgacgcacgcctttgtcactttgtccttgtggcctgttgaaatgccactcctgctttacaaattcaccaactgttgcatgagtcatttccacctcaatgagtaccaggtccttgaggatggggaaaagtaagccaccactgtgggggtcctgggctcctaggtgcagaagaggctccagaaacaggccaggtcgtgggccatgaccccacactagccctctggtccctcacacgggtggattggggggctgtgtcacgggatcttaggatcttcaagacaaagacccaggacaagaacacaagcccactcccattcttcacaggcctcgagaaatctttgggcaatgaagtcagactgtgccaaagcccatgtttctgtctctccaaggcccctggcccccactgcctagcctaggtcaggtcatgtgggcaagcgagcccccacagcctcacagcccctaccccagggccagggcaaactcctgccctgtccccctccattcctgccctccctccttccacaaactgcaccagctggggagaaatccttcagccgacagaatgaggtgaaaatagtgcaattttaggctttgtaactgagattagggcaggtggccacccattctccccttcctcaggccagcctctgacacaatgaccctggaagcctggcagccctccgtaatggtcagcatcctcccctgccatccccaacccacaccatgagctcagccagggcaggggcagcctctgtctcattcaccacagaatccacagaacccagcacagagtatgagctcagtaaattctcctcatacatgactgcactgactggaccgggcacatgctacagggcaacacccacggctcagctggccctggctttggatctcagtcccacctcttcaagctgtccagcgtggggcacatcggctacagccttgccaaatgaaggcttgccaggatgaagaggtgaagacaggacaagcacagtatgtggcacacaggaggcctctgataacatcagtccccttccctaaagacctgggcagtccctgtcactggggcctcacatttcatgtcgagaattcactatttctcagcactgatttcaaataaagccaccaagagtctgacgaggcaacatggcagagttctgagggtggagtgaacaaaaggtcattttttacagaaaactcaggatctcccctctgcacagtgctaaagccctgtctcaaagttcagagcccggaaggtgcagagatgtggcccttggaaatcaagcccttaagaaaacagcccagctgtgtagggccggaagccccaggctgcagtcctgtggtctggaggcagccaatattcaggtgagagatgtgcccagctgccggtgggtccagggggcacggagcccccaccgtccctggcccaggtctaggactaagtcagtgggcccaggccagctccaagggccacagctcctcactcgggggccgcgccggagcagccgcagcagctggggcgccgcagggactgcatgacagcccgcagtggccccctccggccctccacagacaggctgtcctcgctggcgggcgcccgctgcagctgctcaaactgcatctccaggtgcttctggatggccacaccgagcacctccaggtccaccgcagctccgtacacctcccatgtcatgccctcagcatcccatcgcacatcccgcacaggggacggcacctcctccaggctggaccccagagttacctctgggaacacatgcagggctgcaggcgcttccagggacggactggtggccacagccttgcaggccgccactggggccgcctgcacaccagcatcctgggctgacagcggggatgcctctgcaggggccaagtcattggctgaggtcatggtccacacatctttggtcctagagccaggctctgggactaacccagcgggaccccaaaggtgggcacagcaatgggaatgcccagggagccccccagacaacctacagtggatcttcaccccatgctgagcctgcagcccagactcgctcactgacgccactagtttgggaaaggccaggatccctgtggcaggtagggcatggcagcagccaccagccctcacctccctcatgccacagagtagagcagctgggggcagagcatggcaggtggtggtagccagctgttcagcagctttgggctcagcctgggcactgctgctgtgggcagttgtgtcccccaggtctagtggtggcactgacaactgactcgcccccagcatccaggctgagttagaagtctcatcctcaggagccaggtccctttccaggcctgcaggggcctggccaccctggccagaagtaccacctggctgcagctgagccctgtggacagggctgctgccaagggctgagcagctgagactggccttccgagcaccactgtgtccccgcatctgggtgctacggaccaggtctgaatggctcctctgcatagcagcagcactaggggcccgcaggcgacacaggtcactgccgcccatggtggacacattgcccacagtgctgctccaccagtggcctccagcactgggtcgcgccttggggccagaggcccgtgctggcttcatgctctcaggcgggttcccctcttcctccggggcctggggtctggtgctggcctcgcccagctgggcctgccacacggtgctgctggcagtcttgcggagctctggcctctgttcccggccttcacccagcaggctggaagagctctgggacaggggctgaaggcgggggctcaggggtgcccagggacccggctcggggcggctggagctcatggctgcctctagctccaggggcaaggagaggccccatgcatcagctttttccatgagggactcattcagcatctggtcattgattccacagcatctcctgagcccctactgcgtgcccagctgtagggcttaatgttctctctcctgccccatttgatgccgaagttgctatggttgtggccgatgtcccgtggccaatgccaggctgtcctgctgcctcaggttccacctgtcagcaactggaagatcaaccacctctcaaggaccaggcaggaatgcacacagcacaaacccccattgcacagtggggatacagcaccctccaggaggtggtttaatccaccccagagtgaacggggcctgataggaacactcagggccaactctgggcaaagcagcaggcagcattccacgccccgcattgaggtctccgcgccggcggctacccctttcctctcgccttctccatcctagctccgcctctcac

SEQ ID NO: 15498 - RNA, 6557 nt, Homo sapiens
  source 1..6557: mol_type = other RNA
gctgggattacaggcatgagccactgtaccaggctgagtccacacttctaagcttgctgttgctctcagacttgcagaacaacctattaaacagaagtaggtaaaagttgagaaagggaagtggccaccacagaaccagttctgctgagaacgaggactcgagtcaggctatgctaccctccttccatggccatgggaaaaaggggtgtgtgctgttggtgtgagagatctggatcttaacagatcagacttaaactaatttgcccatgatgaccgtgtggatttggagggacctgggaatctcacagacctatgggatgtcccagtgatatgtcctgggcttcataccagccctgccctgcctgacaagttggatgaaaactgataaaggacttgtcatagcttcagatggcaaaaccaggccaggccagaatgaaaaaggagaaggaatttaacatgggcaaatgccaagctctgcatttaactaaccaaggctgcttggcgtgaacaaaactgagacagagcaatgcatggagaaaagggttgggcatttgtgggctacaagcttggcatgacatggatgcaaatgtcaatgggtgcacccccagatgcctgtgactccctctggtggtttctgtgcacaacttcccccaaaataggccctacgactccagcagaaacctaccctggggctcctagagcttcctagcctgcctgccagagagcagaagtgcctggaggctacatcttcacccctgggtagtccttactctgaggtgggactgcatccagggctcccctttagggtctgacttggactgaaatcacaccctgccttgccttctgcccctcccttaacttgctctcccctccctaataactccagcatcctcatctcagcagaagcttctggggaacccagcccaagatgagtggtgagggctagggtagccctcctcaatgcactctgggaactacattttcagaagccccagccagagggccaagtcccaggcagggtgcaaagctgtggggcgaggaacctggaaagaggctctgaacaagggacttttaaggaagtgggatgtgggctgtgatcacagccaagctggcagggtaagaggtggcccctgaatgtggctatgagaggggtgcccaacactaccagcctgtgtgctgagcactaactcagtgccaggcactacttgggttattctatttaatctccacaccaagcatgtgaaggaggcaccattgtcatccccatcttacagatgaggaagatgatcaaggcttgtaacttgcccaagatcacatggctataggtgtggatcctatatatccagattcaaactccagctttagcccactaagctacggtggccaaccccagcccaaagtgttgggacctgcgtgtagaagaccccttcagcccttgtaaagttaggatctagcatgtctaaggggacagagacccaatccaggtgacacaggaggtaagatcacagtggaacaggccatccctgcttttccaccaccaccagcactgtgacctcagaccagctctactctatgagtttcttgtgacagtgatggcagcctggggccagacaagggatgcgtgtcttgtgtcctggacacaagacaggcaggcccagaggggacaagctatatgaagagaggcttcagctgtcgggggtcctgaatgccatggaaggagagcaggtgggcagaagcagggagcccctggagcagacagaggggggattcctgctgaggcaaggggctctaggactccagggtttatgctccaaagaacagaatttaccaggacaaaataaacaagaccagtcaggaccgatgccccatccctgctggggtctggcaaagctctcacctccaaatttgtatctgttttgaattcaaagccaaacaaacacatcaacagtgaactccaacacctcccagagcagggcctgaaagggacccagaaagtctggccagaaatctagagtccaaggggaggagatctgtaaactaaaccgctggccatgctctggggccctaaaccactgcaggcatcagggctgttccaggagagggcacagcaaagggggttgggaggggtctccagttccaatcagaaatgaggctgcagtcacttcaggtagacctgtcagcagcagctgtgcaactgggctagggagacaaggatcgtggtttagccaggagaatcatctggggccccagccaagacacaggtgttggatttcagcaccgctctgcaaatactcatctcagtgacgatgaggtgagtgggagcttggctgagcccagcccggcctgccatcctggcaagccagggcagcatggaggtagcacagagtggcacccagccagcgtgaatgcataagaatctgcacgtgacacagaagaaagtctcttcatgaagtaggtttcactggtcccagccaaaccctgtggcaggtggccctttctgcacctgctgaacatgccattcaccttgacccaggtagtggcctcaccctcctcttgctcaaactggaaacctcagcatcctgaaatgcctcctccccaaatccattgcacacatgtgtgcctgtgtatgcgtgtgtgtgcacgtgtatgaacccagcccccagctgcccactccattgcccctaaacaggcccctccttggtgtcacctggcacatctccactggaagccaaatggatatttctaaactgaaatctggtcccacctcagaaccccttccacagttcccttaaagttcctttcctcatttacatcaggatcttcacaatggggacccctggtcacctcccaacccaacaaacgctccaaatgagccgccactgcagaaactcattatggcccaggcaggacaggcacatccaagtatctgaccaggctgttccatctgccaggcaggtcctgccctctctccacccacctgtctaacccctgcatcctcaagaccctacttagctatggccctgtgtgaaaggtccctccccatgcacccacagccatttgttctctctcatgtggccctaacaggctggggttcctggagactccatggggagccaggcatgaagatggcatatacccatgtgtcactccccagaacgtgagctgcctgccctggcaccatacacaaagggactgacagccccagaatcccaaggggtgcacctatgcatatgggaaaggcatgtttacgggtgagaatggtccatcgttgggcttcaggaggcatctgacctgacgcacgcctttgtcactttgtccttgtggcctgttgaaatgccactcctgctttacaaattcaccaactgttgcatgagtcatttccacctcaatgagtaccaggtccttgaggatggggaaaagtaagccaccactgtgggggtcctgggctcctaggtgcagaagaggctccagaaacaggccaggtcgtgggccatgaccccacactagccctctggtccctcacacgggtggattggggggctgtgtcacgggatcttaggatcttcaagacaaagacccaggacaagaacacaagcccactcccattcttcacaggcctcgagaaatctttgggcaatgaagtcagactgtgccaaagcccatgtttctgtctctccaaggcccctggcccccactgcctagcctaggtcaggtcatgtgggcaagcgagcccccacagcctcacagcccctaccccagggccagggcaaactcctgccctgtccccctccattcctgccctccctccttccacaaactgcaccagctggggagaaatccttcagccgacagaatgaggtgaaaatagtgcaattttaggctttgtaactgagattagggcaggtggccacccattctccccttcctcaggccagcctctgacacaatgaccctggaagcctggcagccctccgtaatggtcagcatcctcccctgccatccccaacccacaccatgagctcagccagggcaggggcagcctctgtctcattcaccacagaatccacagaacccagcacagagtatgagctcagtaaattctcctcatacatgactgcactgactggaccgggcacatgctacagggcaacacccacggctcagctggccctggctttggatctcagtcccacctcttcaagctgtccagcgtggggcacatcggctacagccttgccaaatgaaggcttgccaggatgaagaggtgaagacaggacaagcacagtatgtggcacacaggaggcctctgataacatcagtccccttccctaaagacctgggcagtccctgtcactggggcctcacatttcatgtcgagaattcactatttctcagcactgatttcaaataaagccaccaagagtctgacgaggcaacatggcagagttctgagggtggagtgaacaaaaggtcattttttacagaaaactcaggatctcccctctgcacagtgctaaagccctgtctcaaagttcagagcccggaaggtgcagagatgtggcccttggaaatcaagcccttaagaaaacagcccagctgtgtagggccggaagccccaggctgcagtcctgtggtctggaggcagccaatattcaggtgagagatgtgcccagctgccggtgggtccagggggcacggagcccccaccgtccctggcccaggtctaggactaagtcagtgggcccaggccagctccaagggccacagctcctcactcgggggccgcgccggagcagccgcagcagctggggcgccgcagggactgcatgacagcccgcagtggccccctccggccctccacagacaggctgtcctcgctggcgggcgcccgctgcagctgctcaaactgcatctccaggtgcttctggatggccacaccgagcacctccaggtccaccgcagctccgtacacctcccatgtcatgccctcagcatcccatcgcacatcccgcacaggggacggcacctcctccaggctggaccccagagttacctctgggaacacatgcagggctgcaggcgcttccagggacggactggtggccacagccttgcaggccgccactggggccgcctgcacaccagcatcctgggctgacagcggggatgcctctgcaggggccaagtcattggctgaggtcatggtccacacatctttggtcctagagccaggctctgggactaacccagcgggaccccaaaggtgggcacagcaatgggaatgcccagggagccccccagacaacctacagtggatcttcaccccatgctgagcctgcagcccagactcgctcactgacgccactagtttgggaaaggccaggatccctgtggcaggtagggcatggcagcagccaccagccctcacctccctcatgccacagagtagagcagctgggggcagagcatggcaggtggtggtagccagctgttcagcagctttgggctcagcctgggcactgctgctgtgggcagttgtgtcccccaggtctagtggtggcactgacaactgactcgcccccagcatccaggctgagttagaagtctcatcctcaggagccaggtccctttccaggcctgcaggggcctggccaccctggccagaagtaccacctggctgcagctgagccctgtggacagggctgctgccaagggctgagcagctgagactggccttccgagcaccactgtgtccccgcatctgggtgctacggaccaggtctgaatggctcctctgcatagcagcagcactaggggcccgcaggcgacacaggtcactgccgcccatggtggacacattgcccacagtgctgctccaccagtggcctccagcactgggtcgcgccttggggccagaggcccgtgctggcttcatgctctcaggcgggttcccctcttcctccggggcctggggtctggtgctggcctcgcccagctgggcctgccacacggtgctgctggcagtcttgcggagctctggcctctgttcccggccttcacccagcaggctggaagagctctgggacaggggctgaaggcgggggctcaggggtgcccagggacccggctcggggcggctggagctcatggctgcctgatgtgtcgtcggcactcagaggattatctgctgtgtgcctgaccaagagaacaagcaaatacaagaacacacccacagaggagggcactgagtgccaaaaatggggtctgagggagggcaccaccaaggcaggagagctcacggagggtgagagatgagaaaaggcttcctggaggaccagccacgtaagtcaggccttaatgttctctctcctgccccatttgatgccgaagttgctatggttgtggccgatgtcccgtggccaatgccaggctgtcctgctgcctcaggttccacctgtcagcaactggaagatcaaccaccacgccccgcattgaggtctccgcgccggcggctacccctttcctctcgccttctccatcctagctccgcctctcac

SEQ ID NO: 15499 - RNA, 6342 nt, Homo sapiens
  source 1..6342: mol_type = other RNA
gctgggattacaggcatgagccactgtaccaggctgagtccacacttctaagcttgctgttgctctcagacttgcagaacaacctattaaacagaagtaggtaaaagttgagaaagggaagtggccaccacagaaccagttctgctgagaacgaggactcgagtcaggctatgctaccctccttccatggccatgggaaaaaggggtgtgtgctgttggtgtgagagatctggatcttaacagatcagacttaaactaatttgcccatgatgaccgtgtggatttggagggacctgggaatctcacagacctatgggatgtcccagtgatatgtcctgggcttcataccagccctgccctgcctgacaagttggatgaaaactgataaaggacttgtcatagcttcagatggcaaaaccaggccaggccagaatgaaaaaggagaaggaatttaacatgggcaaatgccaagctctgcatttaactaaccaaggctgcttggcgtgaacaaaactgagacagagcaatgcatggagaaaagggttgggcatttgtgggctacaagcttggcatgacatggatgcaaatgtcaatgggtgcacccccagatgcctgtgactccctctggtggtttctgtgcacaacttcccccaaaataggccctacgactccagcagaaacctaccctggggctcctagagcttcctagcctgcctgccagagagcagaagtgcctggaggctacatcttcacccctgggtagtccttactctgaggtgggactgcatccagggctcccctttagggtctgacttggactgaaatcacaccctgccttgccttctgcccctcccttaacttgctctcccctccctaataactccagcatcctcatctcagcagaagcttctggggaacccagcccaagatgagtggtgagggctagggtagccctcctcaatgcactctgggaactacattttcagaagccccagccagagggccaagtcccaggcagggtgcaaagctgtggggcgaggaacctggaaagaggctctgaacaagggacttttaaggaagtgggatgtgggctgtgatcacagccaagctggcagggtaagaggtggcccctgaatgtggctatgagaggggtgcccaacactaccagcctgtgtgctgagcactaactcagtgccaggcactacttgggttattctatttaatctccacaccaagcatgtgaaggaggcaccattgtcatccccatcttacagatgaggaagatgatcaaggcttgtaacttgcccaagatcacatggctataggtgtggatcctatatatccagattcaaactccagctttagcccactaagctacggtggccaaccccagcccaaagtgttgggacctgcgtgtagaagaccccttcagcccttgtaaagttaggatctagcatgtctaaggggacagagacccaatccaggtgacacaggaggtaagatcacagtggaacaggccatccctgcttttccaccaccaccagcactgtgacctcagaccagctctactctatgagtttcttgtgacagtgatggcagcctggggccagacaagggatgcgtgtcttgtgtcctggacacaagacaggcaggcccagaggggacaagctatatgaagagaggcttcagctgtcgggggtcctgaatgccatggaaggagagcaggtgggcagaagcagggagcccctggagcagacagaggggggattcctgctgaggcaaggggctctaggactccagggtttatgctccaaagaacagaatttaccaggacaaaataaacaagaccagtcaggaccgatgccccatccctgctggggtctggcaaagctctcacctccaaatttgtatctgttttgaattcaaagccaaacaaacacatcaacagtgaactccaacacctcccagagcagggcctgaaagggacccagaaagtctggccagaaatctagagtccaaggggaggagatctgtaaactaaaccgctggccatgctctggggccctaaaccactgcaggcatcagggctgttccaggagagggcacagcaaagggggttgggaggggtctccagttccaatcagaaatgaggctgcagtcacttcaggtagacctgtcagcagcagctgtgcaactgggctagggagacaaggatcgtggtttagccaggagaatcatctggggccccagccaagacacaggtgttggatttcagcaccgctctgcaaatactcatctcagtgacgatgaggtgagtgggagcttggctgagcccagcccggcctgccatcctggcaagccagggcagcatggaggtagcacagagtggcacccagccagcgtgaatgcataagaatctgcacgtgacacagaagaaagtctcttcatgaagtaggtttcactggtcccagccaaaccctgtggcaggtggccctttctgcacctgctgaacatgccattcaccttgacccaggtagtggcctcaccctcctcttgctcaaactggaaacctcagcatcctgaaatgcctcctccccaaatccattgcacacatgtgtgcctgtgtatgcgtgtgtgtgcacgtgtatgaacccagcccccagctgcccactccattgcccctaaacaggcccctccttggtgtcacctggcacatctccactggaagccaaatggatatttctaaactgaaatctggtcccacctcagaaccccttccacagttcccttaaagttcctttcctcatttacatcaggatcttcacaatggggacccctggtcacctcccaacccaacaaacgctccaaatgagccgccactgcagaaactcattatggcccaggcaggacaggcacatccaagtatctgaccaggctgttccatctgccaggcaggtcctgccctctctccacccacctgtctaacccctgcatcctcaagaccctacttagctatggccctgtgtgaaaggtccctccccatgcacccacagccatttgttctctctcatgtggccctaacaggctggggttcctggagactccatggggagccaggcatgaagatggcatatacccatgtgtcactccccagaacgtgagctgcctgccctggcaccatacacaaagggactgacagccccagaatcccaaggggtgcacctatgcatatgggaaaggcatgtttacgggtgagaatggtccatcgttgggcttcaggaggcatctgacctgacgcacgcctttgtcactttgtccttgtggcctgttgaaatgccactcctgctttacaaattcaccaactgttgcatgagtcatttccacctcaatgagtaccaggtccttgaggatggggaaaagtaagccaccactgtgggggtcctgggctcctaggtgcagaagaggctccagaaacaggccaggtcgtgggccatgaccccacactagccctctggtccctcacacgggtggattggggggctgtgtcacgggatcttaggatcttcaagacaaagacccaggacaagaacacaagcccactcccattcttcacaggcctcgagaaatctttgggcaatgaagtcagactgtgccaaagcccatgtttctgtctctccaaggcccctggcccccactgcctagcctaggtcaggtcatgtgggcaagcgagcccccacagcctcacagcccctaccccagggccagggcaaactcctgccctgtccccctccattcctgccctccctccttccacaaactgcaccagctggggagaaatccttcagccgacagaatgaggtgaaaatagtgcaattttaggctttgtaactgagattagggcaggtggccacccattctccccttcctcaggccagcctctgacacaatgaccctggaagcctggcagccctccgtaatggtcagcatcctcccctgccatccccaacccacaccatgagctcagccagggcaggggcagcctctgtctcattcaccacagaatccacagaacccagcacagagtatgagctcagtaaattctcctcatacatgactgcactgactggaccgggcacatgctacagggcaacacccacggctcagctggccctggctttggatctcagtcccacctcttcaagctgtccagcgtggggcacatcggctacagccttgccaaatgaaggcttgccaggatgaagaggtgaagacaggacaagcacagtatgtggcacacaggaggcctctgataacatcagtccccttccctaaagacctgggcagtccctgtcactggggcctcacatttcatgtcgagaattcactatttctcagcactgatttcaaataaagccaccaagagtctgacgaggcaacatggcagagttctgagggtggagtgaacaaaaggtcattttttacagaaaactcaggatctcccctctgcacagtgctaaagccctgtctcaaagttcagagcccggaaggtgcagagatgtggcccttggaaatcaagcccttaagaaaacagcccagctgtgtagggccggaagccccaggctgcagtcctgtggtctggaggcagccaatattcaggtgagagatgtgcccagctgccggtgggtccagggggcacggagcccccaccgtccctggcccaggtctaggactaagtcagtgggcccaggccagctccaagggccacagctcctcactcgggggccgcgccggagcagccgcagcagctggggcgccgcagggactgcatgacagcccgcagtggccccctccggccctccacagacaggctgtcctcgctggcgggcgcccgctgcagctgctcaaactgcatctccaggtgcttctggatggccacaccgagcacctccaggtccaccgcagctccgtacacctcccatgtcatgccctcagcatcccatcgcacatcccgcacaggggacggcacctcctccaggctggaccccagagttacctctgggaacacatgcagggctgcaggcgcttccagggacggactggtggccacagccttgcaggccgccactggggccgcctgcacaccagcatcctgggctgacagcggggatgcctctgcaggggccaagtcattggctgaggtcatggtccacacatctttggtcctagagccaggctctgggactaacccagcgggaccccaaaggtgggcacagcaatgggaatgcccagggagccccccagacaacctacagtggatcttcaccccatgctgagcctgcagcccagactcgctcactgacgccactagtttgggaaaggccaggatccctgtggcaggtagggcatggcagcagccaccagccctcacctccctcatgccacagagtagagcagctgggggcagagcatggcaggtggtggtagccagctgttcagcagctttgggctcagcctgggcactgctgctgtgggcagttgtgtcccccaggtctagtggtggcactgacaactgactcgcccccagcatccaggctgagttagaagtctcatcctcaggagccaggtccctttccaggcctgcaggggcctggccaccctggccagaagtaccacctggctgcagctgagccctgtggacagggctgctgccaagggctgagcagctgagactggccttccgagcaccactgtgtccccgcatctgggtgctacggaccaggtctgaatggctcctctgcatagcagcagcactaggggcccgcaggcgacacaggtcactgccgcccatggtggacacattgcccacagtgctgctccaccagtggcctccagcactgggtcgcgccttggggccagaggcccgtgctggcttcatgctctcaggcgggttcccctcttcctccggggcctggggtctggtgctggcctcgcccagctgggcctgccacacggtgctgctggcagtcttgcggagctctggcctctgttcccggccttcacccagcaggctggaagagctctgggacaggggctgaaggcgggggctcaggggtgcccagggacccggctcggggcggctggagctcatggctgccttaatgttctctctcctgccccatttgatgccgaagttgctatggttgtggccgatgtcccgtggccaatgccaggctgtcctgctgcctcaggttccacctgtcagcaacacgccccgcattgaggtctccgcgccggcggctacccctttcctctcgccttctccatcctagctccgcctctcac

SEQ ID NO: 15500 - RNA, 6433 nt, Homo sapiens
  source 1..6433: mol_type = other RNA
gctgggattacaggcatgagccactgtaccaggctgagtccacacttctaagcttgctgttgctctcagacttgcagaacaacctattaaacagaagtaggtaaaagttgagaaagggaagtggccaccacagaaccagttctgctgagaacgaggactcgagtcaggctatgctaccctccttccatggccatgggaaaaaggggtgtgtgctgttggtgtgagagatctggatcttaacagatcagacttaaactaatttgcccatgatgaccgtgtggatttggagggacctgggaatctcacagacctatgggatgtcccagtgatatgtcctgggcttcataccagccctgccctgcctgacaagttggatgaaaactgataaaggacttgtcatagcttcagatggcaaaaccaggccaggccagaatgaaaaaggagaaggaatttaacatgggcaaatgccaagctctgcatttaactaaccaaggctgcttggcgtgaacaaaactgagacagagcaatgcatggagaaaagggttgggcatttgtgggctacaagcttggcatgacatggatgcaaatgtcaatgggtgcacccccagatgcctgtgactccctctggtggtttctgtgcacaacttcccccaaaataggccctacgactccagcagaaacctaccctggggctcctagagcttcctagcctgcctgccagagagcagaagtgcctggaggctacatcttcacccctgggtagtccttactctgaggtgggactgcatccagggctcccctttagggtctgacttggactgaaatcacaccctgccttgccttctgcccctcccttaacttgctctcccctccctaataactccagcatcctcatctcagcagaagcttctggggaacccagcccaagatgagtggtgagggctagggtagccctcctcaatgcactctgggaactacattttcagaagccccagccagagggccaagtcccaggcagggtgcaaagctgtggggcgaggaacctggaaagaggctctgaacaagggacttttaaggaagtgggatgtgggctgtgatcacagccaagctggcagggtaagaggtggcccctgaatgtggctatgagaggggtgcccaacactaccagcctgtgtgctgagcactaactcagtgccaggcactacttgggttattctatttaatctccacaccaagcatgtgaaggaggcaccattgtcatccccatcttacagatgaggaagatgatcaaggcttgtaacttgcccaagatcacatggctataggtgtggatcctatatatccagattcaaactccagctttagcccactaagctacggtggccaaccccagcccaaagtgttgggacctgcgtgtagaagaccccttcagcccttgtaaagttaggatctagcatgtctaaggggacagagacccaatccaggtgacacaggaggtaagatcacagtggaacaggccatccctgcttttccaccaccaccagcactgtgacctcagaccagctctactctatgagtttcttgtgacagtgatggcagcctggggccagacaagggatgcgtgtcttgtgtcctggacacaagacaggcaggcccagaggggacaagctatatgaagagaggcttcagctgtcgggggtcctgaatgccatggaaggagagcaggtgggcagaagcagggagcccctggagcagacagaggggggattcctgctgaggcaaggggctctaggactccagggtttatgctccaaagaacagaatttaccaggacaaaataaacaagaccagtcaggaccgatgccccatccctgctggggtctggcaaagctctcacctccaaatttgtatctgttttgaattcaaagccaaacaaacacatcaacagtgaactccaacacctcccagagcagggcctgaaagggacccagaaagtctggccagaaatctagagtccaaggggaggagatctgtaaactaaaccgctggccatgctctggggccctaaaccactgcaggcatcagggctgttccaggagagggcacagcaaagggggttgggaggggtctccagttccaatcagaaatgaggctgcagtcacttcaggtagacctgtcagcagcagctgtgcaactgggctagggagacaaggatcgtggtttagccaggagaatcatctggggccccagccaagacacaggtgttggatttcagcaccgctctgcaaatactcatctcagtgacgatgaggtgagtgggagcttggctgagcccagcccggcctgccatcctggcaagccagggcagcatggaggtagcacagagtggcacccagccagcgtgaatgcataagaatctgcacgtgacacagaagaaagtctcttcatgaagtaggtttcactggtcccagccaaaccctgtggcaggtggccctttctgcacctgctgaacatgccattcaccttgacccaggtagtggcctcaccctcctcttgctcaaactggaaacctcagcatcctgaaatgcctcctccccaaatccattgcacacatgtgtgcctgtgtatgcgtgtgtgtgcacgtgtatgaacccagcccccagctgcccactccattgcccctaaacaggcccctccttggtgtcacctggcacatctccactggaagccaaatggatatttctaaactgaaatctggtcccacctcagaaccccttccacagttcccttaaagttcctttcctcatttacatcaggatcttcacaatggggacccctggtcacctcccaacccaacaaacgctccaaatgagccgccactgcagaaactcattatggcccaggcaggacaggcacatccaagtatctgaccaggctgttccatctgccaggcaggtcctgccctctctccacccacctgtctaacccctgcatcctcaagaccctacttagctatggccctgtgtgaaaggtccctccccatgcacccacagccatttgttctctctcatgtggccctaacaggctggggttcctggagactccatggggagccaggcatgaagatggcatatacccatgtgtcactccccagaacgtgagctgcctgccctggcaccatacacaaagggactgacagccccagaatcccaaggggtgcacctatgcatatgggaaaggcatgtttacgggtgagaatggtccatcgttgggcttcaggaggcatctgacctgacgcacgcctttgtcactttgtccttgtggcctgttgaaatgccactcctgctttacaaattcaccaactgttgcatgagtcatttccacctcaatgagtaccaggtccttgaggatggggaaaagtaagccaccactgtgggggtcctgggctcctaggtgcagaagaggctccagaaacaggccaggtcgtgggccatgaccccacactagccctctggtccctcacacgggtggattggggggctgtgtcacgggatcttaggatcttcaagacaaagacccaggacaagaacacaagcccactcccattcttcacaggcctcgagaaatctttgggcaatgaagtcagactgtgccaaagcccatgtttctgtctctccaaggcccctggcccccactgcctagcctaggtcaggtcatgtgggcaagcgagcccccacagcctcacagcccctaccccagggccagggcaaactcctgccctgtccccctccattcctgccctccctccttccacaaactgcaccagctggggagaaatccttcagccgacagaatgaggtgaaaatagtgcaattttaggctttgtaactgagattagggcaggtggccacccattctccccttcctcaggccagcctctgacacaatgaccctggaagcctggcagccctccgtaatggtcagcatcctcccctgccatccccaacccacaccatgagctcagccagggcaggggcagcctctgtctcattcaccacagaatccacagaacccagcacagagtatgagctcagtaaattctcctcatacatgactgcactgactggaccgggcacatgctacagggcaacacccacggctcagctggccctggctttggatctcagtcccacctcttcaagctgtccagcgtggggcacatcggctacagccttgccaaatgaaggcttgccaggatgaagaggtgaagacaggacaagcacagtatgtggcacacaggaggcctctgataacatcagtccccttccctaaagacctgggcagtccctgtcactggggcctcacatttcatgtcgagaattcactatttctcagcactgatttcaaataaagccaccaagagtctgacgaggcaacatggcagagttctgagggtggagtgaacaaaaggtcattttttacagaaaactcaggatctcccctctgcacagtgctaaagccctgtctcaaagttcagagcccggaaggtgcagagatgtggcccttggaaatcaagcccttaagaaaacagcccagctgtgtagggccggaagccccaggctgcagtcctgtggtctggaggcagccaatattcaggtgagagatgtgcccagctgccggtgggtccagggggcacggagcccccaccgtccctggcccaggtctaggactaagtcagtgggcccaggccagctccaagggccacagctcctcactcgggggccgcgccggagcagccgcagcagctggggcgccgcagggactgcatgacagcccgcagtggccccctccggccctccacagacaggctgtcctcgctggcgggcgcccgctgcagctgctcaaactgcatctccaggtgcttctggatggccacaccgagcacctccaggtccaccgcagctccgtacacctcccatgtcatgccctcagcatcccatcgcacatcccgcacaggggacggcacctcctccaggctggaccccagagttacctctgggaacacatgcagggctgcaggcgcttccagggacggactggtggccacagccttgcaggccgccactggggccgcctgcacaccagcatcctgggctgacagcggggatgcctctgcaggggccaagtcattggctgaggtcatggtccacacatctttggtcctagagccaggctctgggactaacccagcgggaccccaaaggtgggcacagcaatgggaatgcccagggagccccccagacaacctacagtggatcttcaccccatgctgagcctgcagcccagactcgctcactgacgccactagtttgggaaaggccaggatccctgtggcaggtagggcatggcagcagccaccagccctcacctccctcatgccacagagtagagcagctgggggcagagcatggcaggtggtggtagccagctgttcagcagctttgggctcagcctgggcactgctgctgtgggcagttgtgtcccccaggtctagtggtggcactgacaactgactcgcccccagcatccaggctgagttagaagtctcatcctcaggagccaggtccctttccaggcctgcaggggcctggccaccctggccagaagtaccacctggctgcagctgagccctgtggacagggctgctgccaagggctgagcagctgagactggccttccgagcaccactgtgtccccgcatctgggtgctacggaccaggtctgaatggctcctctgcatagcagcagcactaggggcccgcaggcgacacaggtcactgccgcccatggtggacacattgcccacagtgctgctccaccagtggcctccagcactgggtcgcgccttggggccagaggcccgtgctggcttcatgctctcaggcgggttcccctcttcctccggggcctggggtctggtgctggcctcgcccagctgggcctgccacacggtgctgctggcagtcttgcggagctctggcctctgttcccggccttcacccagcaggctggaagagctctgggacaggggctgaaggcgggggctcaggggtgcccagggacccggctcggggcggctggagctcatggctgccttaatgttctctctcctgccccatttgatgccgaagttgctatggttgtggccgatgtcccgtggccaatgccaggctgtcctgctgcctcaggttccacctgtcagcaacctccaggaggtggtttaatccaccccagagtgaacggggcctgataggaacactcagggccaactctgggcaaagcagcaggcagcattccacgccccgcattgaggtctccgcgccggcggctacccctttcctctcgccttctccatcctagctccgcctctcac

SEQ ID NO: 15501 - RNA, 6426 nt, Homo sapiens
  source 1..6426: mol_type = other RNA
gctgggattacaggcatgagccactgtaccaggctgagtccacacttctaagcttgctgttgctctcagacttgcagaacaacctattaaacagaagtaggtaaaagttgagaaagggaagtggccaccacagaaccagttctgctgagaacgaggactcgagtcaggctatgctaccctccttccatggccatgggaaaaaggggtgtgtgctgttggtgtgagagatctggatcttaacagatcagacttaaactaatttgcccatgatgaccgtgtggatttggagggacctgggaatctcacagacctatgggatgtcccagtgatatgtcctgggcttcataccagccctgccctgcctgacaagttggatgaaaactgataaaggacttgtcatagcttcagatggcaaaaccaggccaggccagaatgaaaaaggagaaggaatttaacatgggcaaatgccaagctctgcatttaactaaccaaggctgcttggcgtgaacaaaactgagacagagcaatgcatggagaaaagggttgggcatttgtgggctacaagcttggcatgacatggatgcaaatgtcaatgggtgcacccccagatgcctgtgactccctctggtggtttctgtgcacaacttcccccaaaataggccctacgactccagcagaaacctaccctggggctcctagagcttcctagcctgcctgccagagagcagaagtgcctggaggctacatcttcacccctgggtagtccttactctgaggtgggactgcatccagggctcccctttagggtctgacttggactgaaatcacaccctgccttgccttctgcccctcccttaacttgctctcccctccctaataactccagcatcctcatctcagcagaagcttctggggaacccagcccaagatgagtggtgagggctagggtagccctcctcaatgcactctgggaactacattttcagaagccccagccagagggccaagtcccaggcagggtgcaaagctgtggggcgaggaacctggaaagaggctctgaacaagggacttttaaggaagtgggatgtgggctgtgatcacagccaagctggcagggtaagaggtggcccctgaatgtggctatgagaggggtgcccaacactaccagcctgtgtgctgagcactaactcagtgccaggcactacttgggttattctatttaatctccacaccaagcatgtgaaggaggcaccattgtcatccccatcttacagatgaggaagatgatcaaggcttgtaacttgcccaagatcacatggctataggtgtggatcctatatatccagattcaaactccagctttagcccactaagctacggtggccaaccccagcccaaagtgttgggacctgcgtgtagaagaccccttcagcccttgtaaagttaggatctagcatgtctaaggggacagagacccaatccaggtgacacaggaggtaagatcacagtggaacaggccatccctgcttttccaccaccaccagcactgtgacctcagaccagctctactctatgagtttcttgtgacagtgatggcagcctggggccagacaagggatgcgtgtcttgtgtcctggacacaagacaggcaggcccagaggggacaagctatatgaagagaggcttcagctgtcgggggtcctgaatgccatggaaggagagcaggtgggcagaagcagggagcccctggagcagacagaggggggattcctgctgaggcaaggggctctaggactccagggtttatgctccaaagaacagaatttaccaggacaaaataaacaagaccagtcaggaccgatgccccatccctgctggggtctggcaaagctctcacctccaaatttgtatctgttttgaattcaaagccaaacaaacacatcaacagtgaactccaacacctcccagagcagggcctgaaagggacccagaaagtctggccagaaatctagagtccaaggggaggagatctgtaaactaaaccgctggccatgctctggggccctaaaccactgcaggcatcagggctgttccaggagagggcacagcaaagggggttgggaggggtctccagttccaatcagaaatgaggctgcagtcacttcaggtagacctgtcagcagcagctgtgcaactgggctagggagacaaggatcgtggtttagccaggagaatcatctggggccccagccaagacacaggtgttggatttcagcaccgctctgcaaatactcatctcagtgacgatgaggtgagtgggagcttggctgagcccagcccggcctgccatcctggcaagccagggcagcatggaggtagcacagagtggcacccagccagcgtgaatgcataagaatctgcacgtgacacagaagaaagtctcttcatgaagtaggtttcactggtcccagccaaaccctgtggcaggtggccctttctgcacctgctgaacatgccattcaccttgacccaggtagtggcctcaccctcctcttgctcaaactggaaacctcagcatcctgaaatgcctcctccccaaatccattgcacacatgtgtgcctgtgtatgcgtgtgtgtgcacgtgtatgaacccagcccccagctgcccactccattgcccctaaacaggcccctccttggtgtcacctggcacatctccactggaagccaaatggatatttctaaactgaaatctggtcccacctcagaaccccttccacagttcccttaaagttcctttcctcatttacatcaggatcttcacaatggggacccctggtcacctcccaacccaacaaacgctccaaatgagccgccactgcagaaactcattatggcccaggcaggacaggcacatccaagtatctgaccaggctgttccatctgccaggcaggtcctgccctctctccacccacctgtctaacccctgcatcctcaagaccctacttagctatggccctgtgtgaaaggtccctccccatgcacccacagccatttgttctctctcatgtggccctaacaggctggggttcctggagactccatggggagccaggcatgaagatggcatatacccatgtgtcactccccagaacgtgagctgcctgccctggcaccatacacaaagggactgacagccccagaatcccaaggggtgcacctatgcatatgggaaaggcatgtttacgggtgagaatggtccatcgttgggcttcaggaggcatctgacctgacgcacgcctttgtcactttgtccttgtggcctgttgaaatgccactcctgctttacaaattcaccaactgttgcatgagtcatttccacctcaatgagtaccaggtccttgaggatggggaaaagtaagccaccactgtgggggtcctgggctcctaggtgcagaagaggctccagaaacaggccaggtcgtgggccatgaccccacactagccctctggtccctcacacgggtggattggggggctgtgtcacgggatcttaggatcttcaagacaaagacccaggacaagaacacaagcccactcccattcttcacaggcctcgagaaatctttgggcaatgaagtcagactgtgccaaagcccatgtttctgtctctccaaggcccctggcccccactgcctagcctaggtcaggtcatgtgggcaagcgagcccccacagcctcacagcccctaccccagggccagggcaaactcctgccctgtccccctccattcctgccctccctccttccacaaactgcaccagctggggagaaatccttcagccgacagaatgaggtgaaaatagtgcaattttaggctttgtaactgagattagggcaggtggccacccattctccccttcctcaggccagcctctgacacaatgaccctggaagcctggcagccctccgtaatggtcagcatcctcccctgccatccccaacccacaccatgagctcagccagggcaggggcagcctctgtctcattcaccacagaatccacagaacccagcacagagtatgagctcagtaaattctcctcatacatgactgcactgactggaccgggcacatgctacagggcaacacccacggctcagctggccctggctttggatctcagtcccacctcttcaagctgtccagcgtggggcacatcggctacagccttgccaaatgaaggcttgccaggatgaagaggtgaagacaggacaagcacagtatgtggcacacaggaggcctctgataacatcagtccccttccctaaagacctgggcagtccctgtcactggggcctcacatttcatgtcgagaattcactatttctcagcactgatttcaaataaagccaccaagagtctgacgaggcaacatggcagagttctgagggtggagtgaacaaaaggtcattttttacagaaaactcaggatctcccctctgcacagtgctaaagccctgtctcaaagttcagagcccggaaggtgcagagatgtggcccttggaaatcaagcccttaagaaaacagcccagctgtgtagggccggaagccccaggctgcagtcctgtggtctggaggcagccaatattcaggtgagagatgtgcccagctgccggtgggtccagggggcacggagcccccaccgtccctggcccaggtctaggactaagtcagtgggcccaggccagctccaagggccacagctcctcactcgggggccgcgccggagcagccgcagcagctggggcgccgcagggactgcatgacagcccgcagtggccccctccggccctccacagacaggctgtcctcgctggcgggcgcccgctgcagctgctcaaactgcatctccaggtgcttctggatggccacaccgagcacctccaggtccaccgcagctccgtacacctcccatgtcatgccctcagcatcccatcgcacatcccgcacaggggacggcacctcctccaggctggaccccagagttacctctgggaacacatgcagggctgcaggcgcttccagggacggactggtggccacagccttgcaggccgccactggggccgcctgcacaccagcatcctgggctgacagcggggatgcctctgcaggggccaagtcattggctgaggtcatggtccacacatctttggtcctagagccaggctctgggactaacccagcgggaccccaaaggtgggcacagcaatgggaatgcccagggagccccccagacaacctacagtggatcttcaccccatgctgagcctgcagcccagactcgctcactgacgccactagtttgggaaaggccaggatccctgtggcaggtagggcatggcagcagccaccagccctcacctccctcatgccacagagtagagcagctgggggcagagcatggcaggtggtggtagccagctgttcagcagctttgggctcagcctgggcactgctgctgtgggcagttgtgtcccccaggtctagtggtggcactgacaactgactcgcccccagcatccaggctgagttagaagtctcatcctcaggagccaggtccctttccaggcctgcaggggcctggccaccctggccagaagtaccacctggctgcagctgagccctgtggacagggctgctgccaagggctgagcagctgagactggccttccgagcaccactgtgtccccgcatctgggtgctacggaccaggtctgaatggctcctctgcatagcagcagcactaggggcccgcaggcgacacaggtcactgccgcccatggtggacacattgcccacagtgctgctccaccagtggcctccagcactgggtcgcgccttggggccagaggcccgtgctggcttcatgctctcaggcgggttcccctcttcctccggggcctggggtctggtgctggcctcgcccagctgggcctgccacacggtgctgctggcagtcttgcggagctctggcctctgttcccggccttcacccagcaggctggaagagctctgggacaggggctgaaggcgggggctcaggggtgcccagggacccggctcggggcggctggagctcatggctgccttaatgttctctctcctgccccatttgatgccgaagttgctatggttgtggccgatgtcccgtggccaatgccaggctgtcctgctgcctcaggttccacctgtcagcaacctctcgcccgccggggccgcgcaggcgggggaagcgctgctcctgcggccgccacaggtgccaggtgccgcggcccaagatggagccagagccgacctggcctgggcgcgagacgccgcccgccgccgtcggcccggcccgcggagcaagcgccgggtac

SEQ ID NO: 15502 - RNA, 6497 nt, Homo sapiens
  source 1..6497: mol_type = other RNA
gctgggattacaggcatgagccactgtaccaggctgagtccacacttctaagcttgctgttgctctcagacttgcagaacaacctattaaacagaagtaggtaaaagttgagaaagggaagtggccaccacagaaccagttctgctgagaacgaggactcgagtcaggctatgctaccctccttccatggccatgggaaaaaggggtgtgtgctgttggtgtgagagatctggatcttaacagatcagacttaaactaatttgcccatgatgaccgtgtggatttggagggacctgggaatctcacagacctatgggatgtcccagtgatatgtcctgggcttcataccagccctgccctgcctgacaagttggatgaaaactgataaaggacttgtcatagcttcagatggcaaaaccaggccaggccagaatgaaaaaggagaaggaatttaacatgggcaaatgccaagctctgcatttaactaaccaaggctgcttggcgtgaacaaaactgagacagagcaatgcatggagaaaagggttgggcatttgtgggctacaagcttggcatgacatggatgcaaatgtcaatgggtgcacccccagatgcctgtgactccctctggtggtttctgtgcacaacttcccccaaaataggccctacgactccagcagaaacctaccctggggctcctagagcttcctagcctgcctgccagagagcagaagtgcctggaggctacatcttcacccctgggtagtccttactctgaggtgggactgcatccagggctcccctttagggtctgacttggactgaaatcacaccctgccttgccttctgcccctcccttaacttgctctcccctccctaataactccagcatcctcatctcagcagaagcttctggggaacccagcccaagatgagtggtgagggctagggtagccctcctcaatgcactctgggaactacattttcagaagccccagccagagggccaagtcccaggcagggtgcaaagctgtggggcgaggaacctggaaagaggctctgaacaagggacttttaaggaagtgggatgtgggctgtgatcacagccaagctggcagggtaagaggtggcccctgaatgtggctatgagaggggtgcccaacactaccagcctgtgtgctgagcactaactcagtgccaggcactacttgggttattctatttaatctccacaccaagcatgtgaaggaggcaccattgtcatccccatcttacagatgaggaagatgatcaaggcttgtaacttgcccaagatcacatggctataggtgtggatcctatatatccagattcaaactccagctttagcccactaagctacggtggccaaccccagcccaaagtgttgggacctgcgtgtagaagaccccttcagcccttgtaaagttaggatctagcatgtctaaggggacagagacccaatccaggtgacacaggaggtaagatcacagtggaacaggccatccctgcttttccaccaccaccagcactgtgacctcagaccagctctactctatgagtttcttgtgacagtgatggcagcctggggccagacaagggatgcgtgtcttgtgtcctggacacaagacaggcaggcccagaggggacaagctatatgaagagaggcttcagctgtcgggggtcctgaatgccatggaaggagagcaggtgggcagaagcagggagcccctggagcagacagaggggggattcctgctgaggcaaggggctctaggactccagggtttatgctccaaagaacagaatttaccaggacaaaataaacaagaccagtcaggaccgatgccccatccctgctggggtctggcaaagctctcacctccaaatttgtatctgttttgaattcaaagccaaacaaacacatcaacagtgaactccaacacctcccagagcagggcctgaaagggacccagaaagtctggccagaaatctagagtccaaggggaggagatctgtaaactaaaccgctggccatgctctggggccctaaaccactgcaggcatcagggctgttccaggagagggcacagcaaagggggttgggaggggtctccagttccaatcagaaatgaggctgcagtcacttcaggtagacctgtcagcagcagctgtgcaactgggctagggagacaaggatcgtggtttagccaggagaatcatctggggccccagccaagacacaggtgttggatttcagcaccgctctgcaaatactcatctcagtgacgatgaggtgagtgggagcttggctgagcccagcccggcctgccatcctggcaagccagggcagcatggaggtagcacagagtggcacccagccagcgtgaatgcataagaatctgcacgtgacacagaagaaagtctcttcatgaagtaggtttcactggtcccagccaaaccctgtggcaggtggccctttctgcacctgctgaacatgccattcaccttgacccaggtagtggcctcaccctcctcttgctcaaactggaaacctcagcatcctgaaatgcctcctccccaaatccattgcacacatgtgtgcctgtgtatgcgtgtgtgtgcacgtgtatgaacccagcccccagctgcccactccattgcccctaaacaggcccctccttggtgtcacctggcacatctccactggaagccaaatggatatttctaaactgaaatctggtcccacctcagaaccccttccacagttcccttaaagttcctttcctcatttacatcaggatcttcacaatggggacccctggtcacctcccaacccaacaaacgctccaaatgagccgccactgcagaaactcattatggcccaggcaggacaggcacatccaagtatctgaccaggctgttccatctgccaggcaggtcctgccctctctccacccacctgtctaacccctgcatcctcaagaccctacttagctatggccctgtgtgaaaggtccctccccatgcacccacagccatttgttctctctcatgtggccctaacaggctggggttcctggagactccatggggagccaggcatgaagatggcatatacccatgtgtcactccccagaacgtgagctgcctgccctggcaccatacacaaagggactgacagccccagaatcccaaggggtgcacctatgcatatgggaaaggcatgtttacgggtgagaatggtccatcgttgggcttcaggaggcatctgacctgacgcacgcctttgtcactttgtccttgtggcctgttgaaatgccactcctgctttacaaattcaccaactgttgcatgagtcatttccacctcaatgagtaccaggtccttgaggatggggaaaagtaagccaccactgtgggggtcctgggctcctaggtgcagaagaggctccagaaacaggccaggtcgtgggccatgaccccacactagccctctggtccctcacacgggtggattggggggctgtgtcacgggatcttaggatcttcaagacaaagacccaggacaagaacacaagcccactcccattcttcacaggcctcgagaaatctttgggcaatgaagtcagactgtgccaaagcccatgtttctgtctctccaaggcccctggcccccactgcctagcctaggtcaggtcatgtgggcaagcgagcccccacagcctcacagcccctaccccagggccagggcaaactcctgccctgtccccctccattcctgccctccctccttccacaaactgcaccagctggggagaaatccttcagccgacagaatgaggtgaaaatagtgcaattttaggctttgtaactgagattagggcaggtggccacccattctccccttcctcaggccagcctctgacacaatgaccctggaagcctggcagccctccgtaatggtcagcatcctcccctgccatccccaacccacaccatgagctcagccagggcaggggcagcctctgtctcattcaccacagaatccacagaacccagcacagagtatgagctcagtaaattctcctcatacatgactgcactgactggaccgggcacatgctacagggcaacacccacggctcagctggccctggctttggatctcagtcccacctcttcaagctgtccagcgtggggcacatcggctacagccttgccaaatgaaggcttgccaggatgaagaggtgaagacaggacaagcacagtatgtggcacacaggaggcctctgataacatcagtccccttccctaaagacctgggcagtccctgtcactggggcctcacatttcatgtcgagaattcactatttctcagcactgatttcaaataaagccaccaagagtctgacgaggcaacatggcagagttctgagggtggagtgaacaaaaggtcattttttacagaaaactcaggatctcccctctgcacagtgctaaagccctgtctcaaagttcagagcccggaaggtgcagagatgtggcccttggaaatcaagcccttaagaaaacagcccagctgtgtagggccggaagccccaggctgcagtcctgtggtctggaggcagccaatattcaggtgagagatgtgcccagctgccggtgggtccagggggcacggagcccccaccgtccctggcccaggtctaggactaagtcagtgggcccaggccagctccaagggccacagctcctcactcgggggccgcgccggagcagccgcagcagctggggcgccgcagggactgcatgacagcccgcagtggccccctccggccctccacagacaggctgtcctcgctggcgggcgcccgctgcagctgctcaaactgcatctccaggtgcttctggatggccacaccgagcacctccaggtccaccgcagctccgtacacctcccatgtcatgccctcagcatcccatcgcacatcccgcacaggggacggcacctcctccaggctggaccccagagttacctctgggaacacatgcagggctgcaggcgcttccagggacggactggtggccacagccttgcaggccgccactggggccgcctgcacaccagcatcctgggctgacagcggggatgcctctgcaggggccaagtcattggctgaggtcatggtccacacatctttggtcctagagccaggctctgggactaacccagcgggaccccaaaggtgggcacagcaatgggaatgcccagggagccccccagacaacctacagtggatcttcaccccatgctgagcctgcagcccagactcgctcactgacgccactagtttgggaaaggccaggatccctgtggcaggtagggcatggcagcagccaccagccctcacctccctcatgccacagagtagagcagctgggggcagagcatggcaggtggtggtagccagctgttcagcagctttgggctcagcctgggcactgctgctgtgggcagttgtgtcccccaggtctagtggtggcactgacaactgactcgcccccagcatccaggctgagttagaagtctcatcctcaggagccaggtccctttccaggcctgcaggggcctggccaccctggccagaagtaccacctggctgcagctgagccctgtggacagggctgctgccaagggctgagcagctgagactggccttccgagcaccactgtgtccccgcatctgggtgctacggaccaggtctgaatggctcctctgcatagcagcagcactaggggcccgcaggcgacacaggtcactgccgcccatggtggacacattgcccacagtgctgctccaccagtggcctccagcactgggtcgcgccttggggccagaggcccgtgctggcttcatgctctcaggcgggttcccctcttcctccggggcctggggtctggtgctggcctcgcccagctgggcctgccacacggtgctgctggcagtcttgcggagctctggcctctgttcccggccttcacccagcaggctggaagagctctgggacaggggctgaaggcgggggctcaggggtgcccagggacccggctcggggcggctggagctcatggctgccttaatgttctctctcctgccccatttgatgccgaagttgctatggttgtggccgatgtcccgtggccaatgccaggctgtcctgctgcctcaggttccacctgtcagcaactctcaaggaccaggcaggaatgcacacagcacaaacccccattgcacagtggggatacagcaccctccaggaggtggtttaatccaccccagagtgaacggggcctgataggaacactcagggccaactctgggcaaagcagcaggcagcattccacgccccgcattgaggtctccgcgccggcggctacccctttcctctcgccttctccatcctagctccgcctctcac

SEQ ID NO: 15503 - RNA, 6461 nt, Homo sapiens
  source 1..6461: mol_type = other RNA
gctgggattacaggcatgagccactgtaccaggctgagtccacacttctaagcttgctgttgctctcagacttgcagaacaacctattaaacagaagtaggtaaaagttgagaaagggaagtggccaccacagaaccagttctgctgagaacgaggactcgagtcaggctatgctaccctccttccatggccatgggaaaaaggggtgtgtgctgttggtgtgagagatctggatcttaacagatcagacttaaactaatttgcccatgatgaccgtgtggatttggagggacctgggaatctcacagacctatgggatgtcccagtgatatgtcctgggcttcataccagccctgccctgcctgacaagttggatgaaaactgataaaggacttgtcatagcttcagatggcaaaaccaggccaggccagaatgaaaaaggagaaggaatttaacatgggcaaatgccaagctctgcatttaactaaccaaggctgcttggcgtgaacaaaactgagacagagcaatgcatggagaaaagggttgggcatttgtgggctacaagcttggcatgacatggatgcaaatgtcaatgggtgcacccccagatgcctgtgactccctctggtggtttctgtgcacaacttcccccaaaataggccctacgactccagcagaaacctaccctggggctcctagagcttcctagcctgcctgccagagagcagaagtgcctggaggctacatcttcacccctgggtagtccttactctgaggtgggactgcatccagggctcccctttagggtctgacttggactgaaatcacaccctgccttgccttctgcccctcccttaacttgctctcccctccctaataactccagcatcctcatctcagcagaagcttctggggaacccagcccaagatgagtggtgagggctagggtagccctcctcaatgcactctgggaactacattttcagaagccccagccagagggccaagtcccaggcagggtgcaaagctgtggggcgaggaacctggaaagaggctctgaacaagggacttttaaggaagtgggatgtgggctgtgatcacagccaagctggcagggtaagaggtggcccctgaatgtggctatgagaggggtgcccaacactaccagcctgtgtgctgagcactaactcagtgccaggcactacttgggttattctatttaatctccacaccaagcatgtgaaggaggcaccattgtcatccccatcttacagatgaggaagatgatcaaggcttgtaacttgcccaagatcacatggctataggtgtggatcctatatatccagattcaaactccagctttagcccactaagctacggtggccaaccccagcccaaagtgttgggacctgcgtgtagaagaccccttcagcccttgtaaagttaggatctagcatgtctaaggggacagagacccaatccaggtgacacaggaggtaagatcacagtggaacaggccatccctgcttttccaccaccaccagcactgtgacctcagaccagctctactctatgagtttcttgtgacagtgatggcagcctggggccagacaagggatgcgtgtcttgtgtcctggacacaagacaggcaggcccagaggggacaagctatatgaagagaggcttcagctgtcgggggtcctgaatgccatggaaggagagcaggtgggcagaagcagggagcccctggagcagacagaggggggattcctgctgaggcaaggggctctaggactccagggtttatgctccaaagaacagaatttaccaggacaaaataaacaagaccagtcaggaccgatgccccatccctgctggggtctggcaaagctctcacctccaaatttgtatctgttttgaattcaaagccaaacaaacacatcaacagtgaactccaacacctcccagagcagggcctgaaagggacccagaaagtctggccagaaatctagagtccaaggggaggagatctgtaaactaaaccgctggccatgctctggggccctaaaccactgcaggcatcagggctgttccaggagagggcacagcaaagggggttgggaggggtctccagttccaatcagaaatgaggctgcagtcacttcaggtagacctgtcagcagcagctgtgcaactgggctagggagacaaggatcgtggtttagccaggagaatcatctggggccccagccaagacacaggtgttggatttcagcaccgctctgcaaatactcatctcagtgacgatgaggtgagtgggagcttggctgagcccagcccggcctgccatcctggcaagccagggcagcatggaggtagcacagagtggcacccagccagcgtgaatgcataagaatctgcacgtgacacagaagaaagtctcttcatgaagtaggtttcactggtcccagccaaaccctgtggcaggtggccctttctgcacctgctgaacatgccattcaccttgacccaggtagtggcctcaccctcctcttgctcaaactggaaacctcagcatcctgaaatgcctcctccccaaatccattgcacacatgtgtgcctgtgtatgcgtgtgtgtgcacgtgtatgaacccagcccccagctgcccactccattgcccctaaacaggcccctccttggtgtcacctggcacatctccactggaagccaaatggatatttctaaactgaaatctggtcccacctcagaaccccttccacagttcccttaaagttcctttcctcatttacatcaggatcttcacaatggggacccctggtcacctcccaacccaacaaacgctccaaatgagccgccactgcagaaactcattatggcccaggcaggacaggcacatccaagtatctgaccaggctgttccatctgccaggcaggtcctgccctctctccacccacctgtctaacccctgcatcctcaagaccctacttagctatggccctgtgtgaaaggtccctccccatgcacccacagccatttgttctctctcatgtggccctaacaggctggggttcctggagactccatggggagccaggcatgaagatggcatatacccatgtgtcactccccagaacgtgagctgcctgccctggcaccatacacaaagggactgacagccccagaatcccaaggggtgcacctatgcatatgggaaaggcatgtttacgggtgagaatggtccatcgttgggcttcaggaggcatctgacctgacgcacgcctttgtcactttgtccttgtggcctgttgaaatgccactcctgctttacaaattcaccaactgttgcatgagtcatttccacctcaatgagtaccaggtccttgaggatggggaaaagtaagccaccactgtgggggtcctgggctcctaggtgcagaagaggctccagaaacaggccaggtcgtgggccatgaccccacactagccctctggtccctcacacgggtggattggggggctgtgtcacgggatcttaggatcttcaagacaaagacccaggacaagaacacaagcccactcccattcttcacaggcctcgagaaatctttgggcaatgaagtcagactgtgccaaagcccatgtttctgtctctccaaggcccctggcccccactgcctagcctaggtcaggtcatgtgggcaagcgagcccccacagcctcacagcccctaccccagggccagggcaaactcctgccctgtccccctccattcctgccctccctccttccacaaactgcaccagctggggagaaatccttcagccgacagaatgaggtgaaaatagtgcaattttaggctttgtaactgagattagggcaggtggccacccattctccccttcctcaggccagcctctgacacaatgaccctggaagcctggcagccctccgtaatggtcagcatcctcccctgccatccccaacccacaccatgagctcagccagggcaggggcagcctctgtctcattcaccacagaatccacagaacccagcacagagtatgagctcagtaaattctcctcatacatgactgcactgactggaccgggcacatgctacagggcaacacccacggctcagctggccctggctttggatctcagtcccacctcttcaagctgtccagcgtggggcacatcggctacagccttgccaaatgaaggcttgccaggatgaagaggtgaagacaggacaagcacagtatgtggcacacaggaggcctctgataacatcagtccccttccctaaagacctgggcagtccctgtcactggggcctcacatttcatgtcgagaattcactatttctcagcactgatttcaaataaagccaccaagagtctgacgaggcaacatggcagagttctgagggtggagtgaacaaaaggtcattttttacagaaaactcaggatctcccctctgcacagtgctaaagccctgtctcaaagttcagagcccggaaggtgcagagatgtggcccttggaaatcaagcccttaagaaaacagcccagctgtgtagggccggaagccccaggctgcagtcctgtggtctggaggcagccaatattcaggtgagagatgtgcccagctgccggtgggtccagggggcacggagcccccaccgtccctggcccaggtctaggactaagtcagtgggcccaggccagctccaagggccacagctcctcactcgggggccgcgccggagcagccgcagcagctggggcgccgcagggactgcatgacagcccgcagtggccccctccggccctccacagacaggctgtcctcgctggcgggcgcccgctgcagctgctcaaactgcatctccaggtgcttctggatggccacaccgagcacctccaggtccaccgcagctccgtacacctcccatgtcatgccctcagcatcccatcgcacatcccgcacaggggacggcacctcctccaggctggaccccagagttacctctgggaacacatgcagggctgcaggcgcttccagggacggactggtggccacagccttgcaggccgccactggggccgcctgcacaccagcatcctgggctgacagcggggatgcctctgcaggggccaagtcattggctgaggtcatggtccacacatctttggtcctagagccaggctctgggactaacccagcgggaccccaaaggtgggcacagcaatgggaatgcccagggagccccccagacaacctacagtggatcttcaccccatgctgagcctgcagcccagactcgctcactgacgccactagtttgggaaaggccaggatccctgtggcaggtagggcatggcagcagccaccagccctcacctccctcatgccacagagtagagcagctgggggcagagcatggcaggtggtggtagccagctgttcagcagctttgggctcagcctgggcactgctgctgtgggcagttgtgtcccccaggtctagtggtggcactgacaactgactcgcccccagcatccaggctgagttagaagtctcatcctcaggagccaggtccctttccaggcctgcaggggcctggccaccctggccagaagtaccacctggctgcagctgagccctgtggacagggctgctgccaagggctgagcagctgagactggccttccgagcaccactgtgtccccgcatctgggtgctacggaccaggtctgaatggctcctctgcatagcagcagcactaggggcccgcaggcgacacaggtcactgccgcccatggtggacacattgcccacagtgctgctccaccagtggcctccagcactgggtcgcgccttggggccagaggcccgtgctggcttcatgctctcaggcgggttcccctcttcctccggggcctggggtctggtgctggcctcgcccagctgggcctgccacacggtgctgctggcagtcttgcggagctctggcctctgttcccggccttcacccagcaggctggaagagctctgggacaggggctgaaggcgggggctcaggggtgcccagggacccggctcggggcggctggagctcatggctgccttaatgttctctctcctgccccatttgatgccgaagttgctatggttgtggccgatgtcccgtggccaatgccaggctgtcctgctgcctcaggttccacctgtcagcaactctcaaggaccaggcaggaatgcacacagcacaaacccccattgcacagtggggatacagcaccctccaggaggtggtttaatccaccccagagtgaacggggcctgataggaacactcagggccaactctgggcaaagcagcaggcagcattcccctttcctctcgccttctccatcctagctccgcctctcac

SEQ ID NO: 15504 - RNA, 6581 nt, Homo sapiens
  source 1..6581: mol_type = other RNA
gctgggattacaggcatgagccactgtaccaggctgagtccacacttctaagcttgctgttgctctcagacttgcagaacaacctattaaacagaagtaggtaaaagttgagaaagggaagtggccaccacagaaccagttctgctgagaacgaggactcgagtcaggctatgctaccctccttccatggccatgggaaaaaggggtgtgtgctgttggtgtgagagatctggatcttaacagatcagacttaaactaatttgcccatgatgaccgtgtggatttggagggacctgggaatctcacagacctatgggatgtcccagtgatatgtcctgggcttcataccagccctgccctgcctgacaagttggatgaaaactgataaaggacttgtcatagcttcagatggcaaaaccaggccaggccagaatgaaaaaggagaaggaatttaacatgggcaaatgccaagctctgcatttaactaaccaaggctgcttggcgtgaacaaaactgagacagagcaatgcatggagaaaagggttgggcatttgtgggctacaagcttggcatgacatggatgcaaatgtcaatgggtgcacccccagatgcctgtgactccctctggtggtttctgtgcacaacttcccccaaaataggccctacgactccagcagaaacctaccctggggctcctagagcttcctagcctgcctgccagagagcagaagtgcctggaggctacatcttcacccctgggtagtccttactctgaggtgggactgcatccagggctcccctttagggtctgacttggactgaaatcacaccctgccttgccttctgcccctcccttaacttgctctcccctccctaataactccagcatcctcatctcagcagaagcttctggggaacccagcccaagatgagtggtgagggctagggtagccctcctcaatgcactctgggaactacattttcagaagccccagccagagggccaagtcccaggcagggtgcaaagctgtggggcgaggaacctggaaagaggctctgaacaagggacttttaaggaagtgggatgtgggctgtgatcacagccaagctggcagggtaagaggtggcccctgaatgtggctatgagaggggtgcccaacactaccagcctgtgtgctgagcactaactcagtgccaggcactacttgggttattctatttaatctccacaccaagcatgtgaaggaggcaccattgtcatccccatcttacagatgaggaagatgatcaaggcttgtaacttgcccaagatcacatggctataggtgtggatcctatatatccagattcaaactccagctttagcccactaagctacggtggccaaccccagcccaaagtgttgggacctgcgtgtagaagaccccttcagcccttgtaaagttaggatctagcatgtctaaggggacagagacccaatccaggtgacacaggaggtaagatcacagtggaacaggccatccctgcttttccaccaccaccagcactgtgacctcagaccagctctactctatgagtttcttgtgacagtgatggcagcctggggccagacaagggatgcgtgtcttgtgtcctggacacaagacaggcaggcccagaggggacaagctatatgaagagaggcttcagctgtcgggggtcctgaatgccatggaaggagagcaggtgggcagaagcagggagcccctggagcagacagaggggggattcctgctgaggcaaggggctctaggactccagggtttatgctccaaagaacagaatttaccaggacaaaataaacaagaccagtcaggaccgatgccccatccctgctggggtctggcaaagctctcacctccaaatttgtatctgttttgaattcaaagccaaacaaacacatcaacagtgaactccaacacctcccagagcagggcctgaaagggacccagaaagtctggccagaaatctagagtccaaggggaggagatctgtaaactaaaccgctggccatgctctggggccctaaaccactgcaggcatcagggctgttccaggagagggcacagcaaagggggttgggaggggtctccagttccaatcagaaatgaggctgcagtcacttcaggtagacctgtcagcagcagctgtgcaactgggctagggagacaaggatcgtggtttagccaggagaatcatctggggccccagccaagacacaggtgttggatttcagcaccgctctgcaaatactcatctcagtgacgatgaggtgagtgggagcttggctgagcccagcccggcctgccatcctggcaagccagggcagcatggaggtagcacagagtggcacccagccagcgtgaatgcataagaatctgcacgtgacacagaagaaagtctcttcatgaagtaggtttcactggtcccagccaaaccctgtggcaggtggccctttctgcacctgctgaacatgccattcaccttgacccaggtagtggcctcaccctcctcttgctcaaactggaaacctcagcatcctgaaatgcctcctccccaaatccattgcacacatgtgtgcctgtgtatgcgtgtgtgtgcacgtgtatgaacccagcccccagctgcccactccattgcccctaaacaggcccctccttggtgtcacctggcacatctccactggaagccaaatggatatttctaaactgaaatctggtcccacctcagaaccccttccacagttcccttaaagttcctttcctcatttacatcaggatcttcacaatggggacccctggtcacctcccaacccaacaaacgctccaaatgagccgccactgcagaaactcattatggcccaggcaggacaggcacatccaagtatctgaccaggctgttccatctgccaggcaggtcctgccctctctccacccacctgtctaacccctgcatcctcaagaccctacttagctatggccctgtgtgaaaggtccctccccatgcacccacagccatttgttctctctcatgtggccctaacaggctggggttcctggagactccatggggagccaggcatgaagatggcatatacccatgtgtcactccccagaacgtgagctgcctgccctggcaccatacacaaagggactgacagccccagaatcccaaggggtgcacctatgcatatgggaaaggcatgtttacgggtgagaatggtccatcgttgggcttcaggaggcatctgacctgacgcacgcctttgtcactttgtccttgtggcctgttgaaatgccactcctgctttacaaattcaccaactgttgcatgagtcatttccacctcaatgagtaccaggtccttgaggatggggaaaagtaagccaccactgtgggggtcctgggctcctaggtgcagaagaggctccagaaacaggccaggtcgtgggccatgaccccacactagccctctggtccctcacacgggtggattggggggctgtgtcacgggatcttaggatcttcaagacaaagacccaggacaagaacacaagcccactcccattcttcacaggcctcgagaaatctttgggcaatgaagtcagactgtgccaaagcccatgtttctgtctctccaaggcccctggcccccactgcctagcctaggtcaggtcatgtgggcaagcgagcccccacagcctcacagcccctaccccagggccagggcaaactcctgccctgtccccctccattcctgccctccctccttccacaaactgcaccagctggggagaaatccttcagccgacagaatgaggtgaaaatagtgcaattttaggctttgtaactgagattagggcaggtggccacccattctccccttcctcaggccagcctctgacacaatgaccctggaagcctggcagccctccgtaatggtcagcatcctcccctgccatccccaacccacaccatgagctcagccagggcaggggcagcctctgtctcattcaccacagaatccacagaacccagcacagagtatgagctcagtaaattctcctcatacatgactgcactgactggaccgggcacatgctacagggcaacacccacggctcagctggccctggctttggatctcagtcccacctcttcaagctgtccagcgtggggcacatcggctacagccttgccaaatgaaggcttgccaggatgaagaggtgaagacaggacaagcacagtatgtggcacacaggaggcctctgataacatcagtccccttccctaaagacctgggcagtccctgtcactggggcctcacatttcatgtcgagaattcactatttctcagcactgatttcaaataaagccaccaagagtctgacgaggcaacatggcagagttctgagggtggagtgaacaaaaggtcattttttacagaaaactcaggatctcccctctgcacagtgctaaagccctgtctcaaagttcagagcccggaaggtgcagagatgtggcccttggaaatcaagcccttaagaaaacagcccagctgtgtagggccggaagccccaggctgcagtcctgtggtctggaggcagccaatattcaggtgagagatgtgcccagctgccggtgggtccagggggcacggagcccccaccgtccctggcccaggtctaggactaagtcagtgggcccaggccagctccaagggccacagctcctcactcgggggccgcgccggagcagccgcagcagctggggcgccgcagggactgcatgacagcccgcagtggccccctccggccctccacagacaggctgtcctcgctggcgggcgcccgctgcagctgctcaaactgcatctccaggtgcttctggatggccacaccgagcacctccaggtccaccgcagctccgtacacctcccatgtcatgccctcagcatcccatcgcacatcccgcacaggggacggcacctcctccaggctggaccccagagttacctctgggaacacatgcagggctgcaggcgcttccagggacggactggtggccacagccttgcaggccgccactggggccgcctgcacaccagcatcctgggctgacagcggggatgcctctgcaggggccaagtcattggctgaggtcatggtccacacatctttggtcctagagccaggctctgggactaacccagcgggaccccaaaggtgggcacagcaatgggaatgcccagggagccccccagacaacctacagtggatcttcaccccatgctgagcctgcagcccagactcgctcactgacgccactagtttgggaaaggccaggatccctgtggcaggtagggcatggcagcagccaccagccctcacctccctcatgccacagagtagagcagctgggggcagagcatggcaggtggtggtagccagctgttcagcagctttgggctcagcctgggcactgctgctgtgggcagttgtgtcccccaggtctagtggtggcactgacaactgactcgcccccagcatccaggctgagttagaagtctcatcctcaggagccaggtccctttccaggcctgcaggggcctggccaccctggccagaagtaccacctggctgcagctgagccctgtggacagggctgctgccaagggctgagcagctgagactggccttccgagcaccactgtgtccccgcatctgggtgctacggaccaggtctgaatggctcctctgcatagcagcagcactaggggcccgcaggcgacacaggtcactgccgcccatggtggacacattgcccacagtgctgctccaccagtggcctccagcactgggtcgcgccttggggccagaggcccgtgctggcttcatgctctcaggcgggttcccctcttcctccggggcctggggtctggtgctggcctcgcccagctgggcctgccacacggtgctgctggcagtcttgcggagctctggcctctgttcccggccttcacccagcaggctggaagagctctgggacaggggctgaaggcgggggctcaggggtgcccagggacccggctcggggcggctggagctcatggctgccttaatgttctctctcctgccccatttgatgccgaagttgctatggttgtggccgatgtcccgtggccaatgccaggctgtcctgctgcctcaggttccacctgtcagcaactctcaaggaccaggcaggaatgcacacagcacaaacccccattgcacagtggggatacagcaccctccaggaggtggtttaatccaccccagagtgaacggggcctgataggaacactcagggccaactctgggcaaagcagcaggcagcattccctctcgcccgccggggccgcgcaggcgggggaagcgctgctcctgcggccgccacaggtgccaggtgccgcggcccaagatggagccagagccgacctggcctgggcgcgagacgccgcccgccgccgtcggcccggcccgcggagcaagcgccgggtac

SEQ ID NO: 15505 - RNA, 6358 nt, Homo sapiens
  source 1..6358: mol_type = other RNA
gctgggattacaggcatgagccactgtaccaggctgagtccacacttctaagcttgctgttgctctcagacttgcagaacaacctattaaacagaagtaggtaaaagttgagaaagggaagtggccaccacagaaccagttctgctgagaacgaggactcgagtcaggctatgctaccctccttccatggccatgggaaaaaggggtgtgtgctgttggtgtgagagatctggatcttaacagatcagacttaaactaatttgcccatgatgaccgtgtggatttggagggacctgggaatctcacagacctatgggatgtcccagtgatatgtcctgggcttcataccagccctgccctgcctgacaagttggatgaaaactgataaaggacttgtcatagcttcagatggcaaaaccaggccaggccagaatgaaaaaggagaaggaatttaacatgggcaaatgccaagctctgcatttaactaaccaaggctgcttggcgtgaacaaaactgagacagagcaatgcatggagaaaagggttgggcatttgtgggctacaagcttggcatgacatggatgcaaatgtcaatgggtgcacccccagatgcctgtgactccctctggtggtttctgtgcacaacttcccccaaaataggccctacgactccagcagaaacctaccctggggctcctagagcttcctagcctgcctgccagagagcagaagtgcctggaggctacatcttcacccctgggtagtccttactctgaggtgggactgcatccagggctcccctttagggtctgacttggactgaaatcacaccctgccttgccttctgcccctcccttaacttgctctcccctccctaataactccagcatcctcatctcagcagaagcttctggggaacccagcccaagatgagtggtgagggctagggtagccctcctcaatgcactctgggaactacattttcagaagccccagccagagggccaagtcccaggcagggtgcaaagctgtggggcgaggaacctggaaagaggctctgaacaagggacttttaaggaagtgggatgtgggctgtgatcacagccaagctggcagggtaagaggtggcccctgaatgtggctatgagaggggtgcccaacactaccagcctgtgtgctgagcactaactcagtgccaggcactacttgggttattctatttaatctccacaccaagcatgtgaaggaggcaccattgtcatccccatcttacagatgaggaagatgatcaaggcttgtaacttgcccaagatcacatggctataggtgtggatcctatatatccagattcaaactccagctttagcccactaagctacggtggccaaccccagcccaaagtgttgggacctgcgtgtagaagaccccttcagcccttgtaaagttaggatctagcatgtctaaggggacagagacccaatccaggtgacacaggaggtaagatcacagtggaacaggccatccctgcttttccaccaccaccagcactgtgacctcagaccagctctactctatgagtttcttgtgacagtgatggcagcctggggccagacaagggatgcgtgtcttgtgtcctggacacaagacaggcaggcccagaggggacaagctatatgaagagaggcttcagctgtcgggggtcctgaatgccatggaaggagagcaggtgggcagaagcagggagcccctggagcagacagaggggggattcctgctgaggcaaggggctctaggactccagggtttatgctccaaagaacagaatttaccaggacaaaataaacaagaccagtcaggaccgatgccccatccctgctggggtctggcaaagctctcacctccaaatttgtatctgttttgaattcaaagccaaacaaacacatcaacagtgaactccaacacctcccagagcagggcctgaaagggacccagaaagtctggccagaaatctagagtccaaggggaggagatctgtaaactaaaccgctggccatgctctggggccctaaaccactgcaggcatcagggctgttccaggagagggcacagcaaagggggttgggaggggtctccagttccaatcagaaatgaggctgcagtcacttcaggtagacctgtcagcagcagctgtgcaactgggctagggagacaaggatcgtggtttagccaggagaatcatctggggccccagccaagacacaggtgttggatttcagcaccgctctgcaaatactcatctcagtgacgatgaggtgagtgggagcttggctgagcccagcccggcctgccatcctggcaagccagggcagcatggaggtagcacagagtggcacccagccagcgtgaatgcataagaatctgcacgtgacacagaagaaagtctcttcatgaagtaggtttcactggtcccagccaaaccctgtggcaggtggccctttctgcacctgctgaacatgccattcaccttgacccaggtagtggcctcaccctcctcttgctcaaactggaaacctcagcatcctgaaatgcctcctccccaaatccattgcacacatgtgtgcctgtgtatgcgtgtgtgtgcacgtgtatgaacccagcccccagctgcccactccattgcccctaaacaggcccctccttggtgtcacctggcacatctccactggaagccaaatggatatttctaaactgaaatctggtcccacctcagaaccccttccacagttcccttaaagttcctttcctcatttacatcaggatcttcacaatggggacccctggtcacctcccaacccaacaaacgctccaaatgagccgccactgcagaaactcattatggcccaggcaggacaggcacatccaagtatctgaccaggctgttccatctgccaggcaggtcctgccctctctccacccacctgtctaacccctgcatcctcaagaccctacttagctatggccctgtgtgaaaggtccctccccatgcacccacagccatttgttctctctcatgtggccctaacaggctggggttcctggagactccatggggagccaggcatgaagatggcatatacccatgtgtcactccccagaacgtgagctgcctgccctggcaccatacacaaagggactgacagccccagaatcccaaggggtgcacctatgcatatgggaaaggcatgtttacgggtgagaatggtccatcgttgggcttcaggaggcatctgacctgacgcacgcctttgtcactttgtccttgtggcctgttgaaatgccactcctgctttacaaattcaccaactgttgcatgagtcatttccacctcaatgagtaccaggtccttgaggatggggaaaagtaagccaccactgtgggggtcctgggctcctaggtgcagaagaggctccagaaacaggccaggtcgtgggccatgaccccacactagccctctggtccctcacacgggtggattggggggctgtgtcacgggatcttaggatcttcaagacaaagacccaggacaagaacacaagcccactcccattcttcacaggcctcgagaaatctttgggcaatgaagtcagactgtgccaaagcccatgtttctgtctctccaaggcccctggcccccactgcctagcctaggtcaggtcatgtgggcaagcgagcccccacagcctcacagcccctaccccagggccagggcaaactcctgccctgtccccctccattcctgccctccctccttccacaaactgcaccagctggggagaaatccttcagccgacagaatgaggtgaaaatagtgcaattttaggctttgtaactgagattagggcaggtggccacccattctccccttcctcaggccagcctctgacacaatgaccctggaagcctggcagccctccgtaatggtcagcatcctcccctgccatccccaacccacaccatgagctcagccagggcaggggcagcctctgtctcattcaccacagaatccacagaacccagcacagagtatgagctcagtaaattctcctcatacatgactgcactgactggaccgggcacatgctacagggcaacacccacggctcagctggccctggctttggatctcagtcccacctcttcaagctgtccagcgtggggcacatcggctacagccttgccaaatgaaggcttgccaggatgaagaggtgaagacaggacaagcacagtatgtggcacacaggaggcctctgataacatcagtccccttccctaaagacctgggcagtccctgtcactggggcctcacatttcatgtcgagaattcactatttctcagcactgatttcaaataaagccaccaagagtctgacgaggcaacatggcagagttctgagggtggagtgaacaaaaggtcattttttacagaaaactcaggatctcccctctgcacagtgctaaagccctgtctcaaagttcagagcccggaaggtgcagagatgtggcccttggaaatcaagcccttaagaaaacagcccagctgtgtagggccggaagccccaggctgcagtcctgtggtctggaggcagccaatattcaggtgagagatgtgcccagctgccggtgggtccagggggcacggagcccccaccgtccctggcccaggtctaggactaagtcagtgggcccaggccagctccaagggccacagctcctcactcgggggccgcgccggagcagccgcagcagctggggcgccgcagggactgcatgacagcccgcagtggccccctccggccctccacagacaggctgtcctcgctggcgggcgcccgctgcagctgctcaaactgcatctccaggtgcttctggatggccacaccgagcacctccaggtccaccgcagctccgtacacctcccatgtcatgccctcagcatcccatcgcacatcccgcacaggggacggcacctcctccaggctggaccccagagttacctctgggaacacatgcagggctgcaggcgcttccagggacggactggtggccacagccttgcaggccgccactggggccgcctgcacaccagcatcctgggctgacagcggggatgcctctgcaggggccaagtcattggctgaggtcatggtccacacatctttggtcctagagccaggctctgggactaacccagcgggaccccaaaggtgggcacagcaatgggaatgcccagggagccccccagacaacctacagtggatcttcaccccatgctgagcctgcagcccagactcgctcactgacgccactagtttgggaaaggccaggatccctgtggcaggtagggcatggcagcagccaccagccctcacctccctcatgccacagagtagagcagctgggggcagagcatggcaggtggtggtagccagctgttcagcagctttgggctcagcctgggcactgctgctgtgggcagttgtgtcccccaggtctagtggtggcactgacaactgactcgcccccagcatccaggctgagttagaagtctcatcctcaggagccaggtccctttccaggcctgcaggggcctggccaccctggccagaagtaccacctggctgcagctgagccctgtggacagggctgctgccaagggctgagcagctgagactggccttccgagcaccactgtgtccccgcatctgggtgctacggaccaggtctgaatggctcctctgcatagcagcagcactaggggcccgcaggcgacacaggtcactgccgcccatggtggacacattgcccacagtgctgctccaccagtggcctccagcactgggtcgcgccttggggccagaggcccgtgctggcttcatgctctcaggcgggttcccctcttcctccggggcctggggtctggtgctggcctcgcccagctgggcctgccacacggtgctgctggcagtcttgcggagctctggcctctgttcccggccttcacccagcaggctggaagagctctgggacaggggctgaaggcgggggctcaggggtgcccagggacccggctcggggcggctggagctcatggctgccttaatgttctctctcctgccccatttgatgccgaagttgctatggttgtggccgatgtcccgtggccaatgccaggctgtcctgctgcctcaggttccacctgtcagcaactggaagatcaaccaccacgccccgcattgaggtctccgcgccggcggctacccctttcctctcgccttctccatcctagctccgcctctcac

SEQ ID NO: 15506 - RNA, 6513 nt, Homo sapiens
  source 1..6513: mol_type = other RNA
gctgggattacaggcatgagccactgtaccaggctgagtccacacttctaagcttgctgttgctctcagacttgcagaacaacctattaaacagaagtaggtaaaagttgagaaagggaagtggccaccacagaaccagttctgctgagaacgaggactcgagtcaggctatgctaccctccttccatggccatgggaaaaaggggtgtgtgctgttggtgtgagagatctggatcttaacagatcagacttaaactaatttgcccatgatgaccgtgtggatttggagggacctgggaatctcacagacctatgggatgtcccagtgatatgtcctgggcttcataccagccctgccctgcctgacaagttggatgaaaactgataaaggacttgtcatagcttcagatggcaaaaccaggccaggccagaatgaaaaaggagaaggaatttaacatgggcaaatgccaagctctgcatttaactaaccaaggctgcttggcgtgaacaaaactgagacagagcaatgcatggagaaaagggttgggcatttgtgggctacaagcttggcatgacatggatgcaaatgtcaatgggtgcacccccagatgcctgtgactccctctggtggtttctgtgcacaacttcccccaaaataggccctacgactccagcagaaacctaccctggggctcctagagcttcctagcctgcctgccagagagcagaagtgcctggaggctacatcttcacccctgggtagtccttactctgaggtgggactgcatccagggctcccctttagggtctgacttggactgaaatcacaccctgccttgccttctgcccctcccttaacttgctctcccctccctaataactccagcatcctcatctcagcagaagcttctggggaacccagcccaagatgagtggtgagggctagggtagccctcctcaatgcactctgggaactacattttcagaagccccagccagagggccaagtcccaggcagggtgcaaagctgtggggcgaggaacctggaaagaggctctgaacaagggacttttaaggaagtgggatgtgggctgtgatcacagccaagctggcagggtaagaggtggcccctgaatgtggctatgagaggggtgcccaacactaccagcctgtgtgctgagcactaactcagtgccaggcactacttgggttattctatttaatctccacaccaagcatgtgaaggaggcaccattgtcatccccatcttacagatgaggaagatgatcaaggcttgtaacttgcccaagatcacatggctataggtgtggatcctatatatccagattcaaactccagctttagcccactaagctacggtggccaaccccagcccaaagtgttgggacctgcgtgtagaagaccccttcagcccttgtaaagttaggatctagcatgtctaaggggacagagacccaatccaggtgacacaggaggtaagatcacagtggaacaggccatccctgcttttccaccaccaccagcactgtgacctcagaccagctctactctatgagtttcttgtgacagtgatggcagcctggggccagacaagggatgcgtgtcttgtgtcctggacacaagacaggcaggcccagaggggacaagctatatgaagagaggcttcagctgtcgggggtcctgaatgccatggaaggagagcaggtgggcagaagcagggagcccctggagcagacagaggggggattcctgctgaggcaaggggctctaggactccagggtttatgctccaaagaacagaatttaccaggacaaaataaacaagaccagtcaggaccgatgccccatccctgctggggtctggcaaagctctcacctccaaatttgtatctgttttgaattcaaagccaaacaaacacatcaacagtgaactccaacacctcccagagcagggcctgaaagggacccagaaagtctggccagaaatctagagtccaaggggaggagatctgtaaactaaaccgctggccatgctctggggccctaaaccactgcaggcatcagggctgttccaggagagggcacagcaaagggggttgggaggggtctccagttccaatcagaaatgaggctgcagtcacttcaggtagacctgtcagcagcagctgtgcaactgggctagggagacaaggatcgtggtttagccaggagaatcatctggggccccagccaagacacaggtgttggatttcagcaccgctctgcaaatactcatctcagtgacgatgaggtgagtgggagcttggctgagcccagcccggcctgccatcctggcaagccagggcagcatggaggtagcacagagtggcacccagccagcgtgaatgcataagaatctgcacgtgacacagaagaaagtctcttcatgaagtaggtttcactggtcccagccaaaccctgtggcaggtggccctttctgcacctgctgaacatgccattcaccttgacccaggtagtggcctcaccctcctcttgctcaaactggaaacctcagcatcctgaaatgcctcctccccaaatccattgcacacatgtgtgcctgtgtatgcgtgtgtgtgcacgtgtatgaacccagcccccagctgcccactccattgcccctaaacaggcccctccttggtgtcacctggcacatctccactggaagccaaatggatatttctaaactgaaatctggtcccacctcagaaccccttccacagttcccttaaagttcctttcctcatttacatcaggatcttcacaatggggacccctggtcacctcccaacccaacaaacgctccaaatgagccgccactgcagaaactcattatggcccaggcaggacaggcacatccaagtatctgaccaggctgttccatctgccaggcaggtcctgccctctctccacccacctgtctaacccctgcatcctcaagaccctacttagctatggccctgtgtgaaaggtccctccccatgcacccacagccatttgttctctctcatgtggccctaacaggctggggttcctggagactccatggggagccaggcatgaagatggcatatacccatgtgtcactccccagaacgtgagctgcctgccctggcaccatacacaaagggactgacagccccagaatcccaaggggtgcacctatgcatatgggaaaggcatgtttacgggtgagaatggtccatcgttgggcttcaggaggcatctgacctgacgcacgcctttgtcactttgtccttgtggcctgttgaaatgccactcctgctttacaaattcaccaactgttgcatgagtcatttccacctcaatgagtaccaggtccttgaggatggggaaaagtaagccaccactgtgggggtcctgggctcctaggtgcagaagaggctccagaaacaggccaggtcgtgggccatgaccccacactagccctctggtccctcacacgggtggattggggggctgtgtcacgggatcttaggatcttcaagacaaagacccaggacaagaacacaagcccactcccattcttcacaggcctcgagaaatctttgggcaatgaagtcagactgtgccaaagcccatgtttctgtctctccaaggcccctggcccccactgcctagcctaggtcaggtcatgtgggcaagcgagcccccacagcctcacagcccctaccccagggccagggcaaactcctgccctgtccccctccattcctgccctccctccttccacaaactgcaccagctggggagaaatccttcagccgacagaatgaggtgaaaatagtgcaattttaggctttgtaactgagattagggcaggtggccacccattctccccttcctcaggccagcctctgacacaatgaccctggaagcctggcagccctccgtaatggtcagcatcctcccctgccatccccaacccacaccatgagctcagccagggcaggggcagcctctgtctcattcaccacagaatccacagaacccagcacagagtatgagctcagtaaattctcctcatacatgactgcactgactggaccgggcacatgctacagggcaacacccacggctcagctggccctggctttggatctcagtcccacctcttcaagctgtccagcgtggggcacatcggctacagccttgccaaatgaaggcttgccaggatgaagaggtgaagacaggacaagcacagtatgtggcacacaggaggcctctgataacatcagtccccttccctaaagacctgggcagtccctgtcactggggcctcacatttcatgtcgagaattcactatttctcagcactgatttcaaataaagccaccaagagtctgacgaggcaacatggcagagttctgagggtggagtgaacaaaaggtcattttttacagaaaactcaggatctcccctctgcacagtgctaaagccctgtctcaaagttcagagcccggaaggtgcagagatgtggcccttggaaatcaagcccttaagaaaacagcccagctgtgtagggccggaagccccaggctgcagtcctgtggtctggaggcagccaatattcaggtgagagatgtgcccagctgccggtgggtccagggggcacggagcccccaccgtccctggcccaggtctaggactaagtcagtgggcccaggccagctccaagggccacagctcctcactcgggggccgcgccggagcagccgcagcagctggggcgccgcagggactgcatgacagcccgcagtggccccctccggccctccacagacaggctgtcctcgctggcgggcgcccgctgcagctgctcaaactgcatctccaggtgcttctggatggccacaccgagcacctccaggtccaccgcagctccgtacacctcccatgtcatgccctcagcatcccatcgcacatcccgcacaggggacggcacctcctccaggctggaccccagagttacctctgggaacacatgcagggctgcaggcgcttccagggacggactggtggccacagccttgcaggccgccactggggccgcctgcacaccagcatcctgggctgacagcggggatgcctctgcaggggccaagtcattggctgaggtcatggtccacacatctttggtcctagagccaggctctgggactaacccagcgggaccccaaaggtgggcacagcaatgggaatgcccagggagccccccagacaacctacagtggatcttcaccccatgctgagcctgcagcccagactcgctcactgacgccactagtttgggaaaggccaggatccctgtggcaggtagggcatggcagcagccaccagccctcacctccctcatgccacagagtagagcagctgggggcagagcatggcaggtggtggtagccagctgttcagcagctttgggctcagcctgggcactgctgctgtgggcagttgtgtcccccaggtctagtggtggcactgacaactgactcgcccccagcatccaggctgagttagaagtctcatcctcaggagccaggtccctttccaggcctgcaggggcctggccaccctggccagaagtaccacctggctgcagctgagccctgtggacagggctgctgccaagggctgagcagctgagactggccttccgagcaccactgtgtccccgcatctgggtgctacggaccaggtctgaatggctcctctgcatagcagcagcactaggggcccgcaggcgacacaggtcactgccgcccatggtggacacattgcccacagtgctgctccaccagtggcctccagcactgggtcgcgccttggggccagaggcccgtgctggcttcatgctctcaggcgggttcccctcttcctccggggcctggggtctggtgctggcctcgcccagctgggcctgccacacggtgctgctggcagtcttgcggagctctggcctctgttcccggccttcacccagcaggctggaagagctctgggacaggggctgaaggcgggggctcaggggtgcccagggacccggctcggggcggctggagctcatggctgccttaatgttctctctcctgccccatttgatgccgaagttgctatggttgtggccgatgtcccgtggccaatgccaggctgtcctgctgcctcaggttccacctgtcagcaactggaagatcaaccacctctcaaggaccaggcaggaatgcacacagcacaaacccccattgcacagtggggatacagcaccctccaggaggtggtttaatccaccccagagtgaacggggcctgataggaacactcagggccaactctgggcaaagcagcaggcagcattccacgccccgcattgaggtctccgcgccggcggctacccctttcctctcgccttctccatcctagctccgcctctcac

SEQ ID NO: 15507 - RNA, 6628 nt, Homo sapiens
  source 1..6628: mol_type = other RNA
gctgggattacaggcatgagccactgtaccaggctgagtccacacttctaagcttgctgttgctctcagacttgcagaacaacctattaaacagaagtaggtaaaagttgagaaagggaagtggccaccacagaaccagttctgctgagaacgaggactcgagtcaggctatgctaccctccttccatggccatgggaaaaaggggtgtgtgctgttggtgtgagagatctggatcttaacagatcagacttaaactaatttgcccatgatgaccgtgtggatttggagggacctgggaatctcacagacctatgggatgtcccagtgatatgtcctgggcttcataccagccctgccctgcctgacaagttggatgaaaactgataaaggacttgtcatagcttcagatggcaaaaccaggccaggccagaatgaaaaaggagaaggaatttaacatgggcaaatgccaagctctgcatttaactaaccaaggctgcttggcgtgaacaaaactgagacagagcaatgcatggagaaaagggttgggcatttgtgggctacaagcttggcatgacatggatgcaaatgtcaatgggtgcacccccagatgcctgtgactccctctggtggtttctgtgcacaacttcccccaaaataggccctacgactccagcagaaacctaccctggggctcctagagcttcctagcctgcctgccagagagcagaagtgcctggaggctacatcttcacccctgggtagtccttactctgaggtgggactgcatccagggctcccctttagggtctgacttggactgaaatcacaccctgccttgccttctgcccctcccttaacttgctctcccctccctaataactccagcatcctcatctcagcagaagcttctggggaacccagcccaagatgagtggtgagggctagggtagccctcctcaatgcactctgggaactacattttcagaagccccagccagagggccaagtcccaggcagggtgcaaagctgtggggcgaggaacctggaaagaggctctgaacaagggacttttaaggaagtgggatgtgggctgtgatcacagccaagctggcagggtaagaggtggcccctgaatgtggctatgagaggggtgcccaacactaccagcctgtgtgctgagcactaactcagtgccaggcactacttgggttattctatttaatctccacaccaagcatgtgaaggaggcaccattgtcatccccatcttacagatgaggaagatgatcaaggcttgtaacttgcccaagatcacatggctataggtgtggatcctatatatccagattcaaactccagctttagcccactaagctacggtggccaaccccagcccaaagtgttgggacctgcgtgtagaagaccccttcagcccttgtaaagttaggatctagcatgtctaaggggacagagacccaatccaggtgacacaggaggtaagatcacagtggaacaggccatccctgcttttccaccaccaccagcactgtgacctcagaccagctctactctatgagtttcttgtgacagtgatggcagcctggggccagacaagggatgcgtgtcttgtgtcctggacacaagacaggcaggcccagaggggacaagctatatgaagagaggcttcagctgtcgggggtcctgaatgccatggaaggagagcaggtgggcagaagcagggagcccctggagcagacagaggggggattcctgctgaggcaaggggctctaggactccagggtttatgctccaaagaacagaatttaccaggacaaaataaacaagaccagtcaggaccgatgccccatccctgctggggtctggcaaagctctcacctccaaatttgtatctgttttgaattcaaagccaaacaaacacatcaacagtgaactccaacacctcccagagcagggcctgaaagggacccagaaagtctggccagaaatctagagtccaaggggaggagatctgtaaactaaaccgctggccatgctctggggccctaaaccactgcaggcatcagggctgttccaggagagggcacagcaaagggggttgggaggggtctccagttccaatcagaaatgaggctgcagtcacttcaggtagacctgtcagcagcagctgtgcaactgggctagggagacaaggatcgtggtttagccaggagaatcatctggggccccagccaagacacaggtgttggatttcagcaccgctctgcaaatactcatctcagtgacgatgaggtgagtgggagcttggctgagcccagcccggcctgccatcctggcaagccagggcagcatggaggtagcacagagtggcacccagccagcgtgaatgcataagaatctgcacgtgacacagaagaaagtctcttcatgaagtaggtttcactggtcccagccaaaccctgtggcaggtggccctttctgcacctgctgaacatgccattcaccttgacccaggtagtggcctcaccctcctcttgctcaaactggaaacctcagcatcctgaaatgcctcctccccaaatccattgcacacatgtgtgcctgtgtatgcgtgtgtgtgcacgtgtatgaacccagcccccagctgcccactccattgcccctaaacaggcccctccttggtgtcacctggcacatctccactggaagccaaatggatatttctaaactgaaatctggtcccacctcagaaccccttccacagttcccttaaagttcctttcctcatttacatcaggatcttcacaatggggacccctggtcacctcccaacccaacaaacgctccaaatgagccgccactgcagaaactcattatggcccaggcaggacaggcacatccaagtatctgaccaggctgttccatctgccaggcaggtcctgccctctctccacccacctgtctaacccctgcatcctcaagaccctacttagctatggccctgtgtgaaaggtccctccccatgcacccacagccatttgttctctctcatgtggccctaacaggctggggttcctggagactccatggggagccaggcatgaagatggcatatacccatgtgtcactccccagaacgtgagctgcctgccctggcaccatacacaaagggactgacagccccagaatcccaaggggtgcacctatgcatatgggaaaggcatgtttacgggtgagaatggtccatcgttgggcttcaggaggcatctgacctgacgcacgcctttgtcactttgtccttgtggcctgttgaaatgccactcctgctttacaaattcaccaactgttgcatgagtcatttccacctcaatgagtaccaggtccttgaggatggggaaaagtaagccaccactgtgggggtcctgggctcctaggtgcagaagaggctccagaaacaggccaggtcgtgggccatgaccccacactagccctctggtccctcacacgggtggattggggggctgtgtcacgggatcttaggatcttcaagacaaagacccaggacaagaacacaagcccactcccattcttcacaggcctcgagaaatctttgggcaatgaagtcagactgtgccaaagcccatgtttctgtctctccaaggcccctggcccccactgcctagcctaggtcaggtcatgtgggcaagcgagcccccacagcctcacagcccctaccccagggccagggcaaactcctgccctgtccccctccattcctgccctccctccttccacaaactgcaccagctggggagaaatccttcagccgacagaatgaggtgaaaatagtgcaattttaggctttgtaactgagattagggcaggtggccacccattctccccttcctcaggccagcctctgacacaatgaccctggaagcctggcagccctccgtaatggtcagcatcctcccctgccatccccaacccacaccatgagctcagccagggcaggggcagcctctgtctcattcaccacagaatccacagaacccagcacagagtatgagctcagtaaattctcctcatacatgactgcactgactggaccgggcacatgctacagggcaacacccacggctcagctggccctggctttggatctcagtcccacctcttcaagctgtccagcgtggggcacatcggctacagccttgccaaatgaaggcttgccaggatgaagaggtgaagacaggacaagcacagtatgtggcacacaggaggcctctgataacatcagtccccttccctaaagacctgggcagtccctgtcactggggcctcacatttcatgtcgagaattcactatttctcagcactgatttcaaataaagccaccaagagtctgacgaggcaacatggcagagttctgagggtggagtgaacaaaaggtcattttttacagaaaactcaggatctcccctctgcacagtgctaaagccctgtctcaaagttcagagcccggaaggtgcagagatgtggcccttggaaatcaagcccttaagaaaacagcccagctgtgtagggccggaagccccaggctgcagtcctgtggtctggaggcagccaatattcaggtgagagatgtgcccagctgccggtgggtccagggggcacggagcccccaccgtccctggcccaggtctaggactaagtcagtgggcccaggccagctccaagggccacagctcctcactcgggggccgcgccggagcagccgcagcagctggggcgccgcagggactgcatgacagcccgcagtggccccctccggccctccacagacaggctgtcctcgctggcgggcgcccgctgcagctgctcaaactgcatctccaggtgcttctggatggccacaccgagcacctccaggtccaccgcagctccgtacacctcccatgtcatgccctcagcatcccatcgcacatcccgcacaggggacggcacctcctccaggctggaccccagagttacctctgggaacacatgcagggctgcaggcgcttccagggacggactggtggccacagccttgcaggccgccactggggccgcctgcacaccagcatcctgggctgacagcggggatgcctctgcaggggccaagtcattggctgaggtcatggtccacacatctttggtcctagagccaggctctgggactaacccagcgggaccccaaaggtgggcacagcaatgggaatgcccagggagccccccagacaacctacagtggatcttcaccccatgctgagcctgcagcccagactcgctcactgacgccactagtttgggaaaggccaggatccctgtggcaggtagggcatggcagcagccaccagccctcacctccctcatgccacagagtagagcagctgggggcagagcatggcaggtggtggtagccagctgttcagcagctttgggctcagcctgggcactgctgctgtgggcagttgtgtcccccaggtctagtggtggcactgacaactgactcgcccccagcatccaggctgagttagaagtctcatcctcaggagccaggtccctttccaggcctgcaggggcctggccaccctggccagaagtaccacctggctgcagctgagccctgtggacagggctgctgccaagggctgagcagctgagactggccttccgagcaccactgtgtccccgcatctgggtgctacggaccaggtctgaatggctcctctgcatagcagcagcactaggggcccgcaggcgacacaggtcactgccgcccatggtggacacattgcccacagtgctgctccaccagtggcctccagcactgggtcgcgccttggggccagaggcccgtgctggcttcatgctctcaggcgggttcccctcttcctccggggcctggggtctggtgctggcctcgcccagctgggcctgccacacggtgctgctggcagtcttgcggagctctggcctctgttcccggccttcacccagcaggctggaagagctctgggacaggggctgaaggcgggggctcaggggtgcccagggacccggctcggggcggctggagctcatggctgccttaatgttctctctcctgccccatttgatgccgaagttgctatggttgtggccgatgtcccgtggccaatgccaggctgtcctgctgcctcaggttccacctgtcagcaacttctcaggagcaaaggcagcgactgcaggcaaatggggctgtgggccggggtaatgatgcgggacaggagaagccaaagggcagcaaggctgggggcggggtaggcggcgcagtaggctgagggaggggaaaaggaagaaggggagagggaggagcgatggcagcaggggtggaggccgaaggagacagggtcccggacagacttgtgaaaatgggaggatgggcagaggagacgtagaagaggggacaggacaggacaatgagaggcggagcgcggggagtgcgatgcggccaccgggggctctgggcgctgggcaggggccaggatgccgggggtctgagcgcaggcagcgggaaggagt

SEQ ID NO: 15508 - RNA, 13347 nt, Homo sapiens
  source 1..13347: mol_type = other RNA
gctgggattacaggcatgagccactgtacccagccaaaatggttactatatattttgaacattatattgcactgtcatcaatagattcgaaaatagttttaccaaattacaggcttagtcttttatagctgtctatatcaatattatttaaagattgagtaccaaagggggcaggaattggaatgtattatctagagcacagaatagtaaataatcaggaaaagggccgggcgcggtggctcatgcctataatcccagcactttgggaggccaaggtgggcggatcacgaggtcagtagatcgagaccatcctggctaacacggtgaaaccccgtctctactaaaaaaataccaaaaattagccgggcgaggtggcaggcgcctatagtcccagctactcgggaggctgaggcaggagaatggcgtgaaccccggggggcggagcctgcagtgagccgagatcgtgccactgcactccagcctgggcaacagcgagactccgtctcaaaaaaaaagaaaaaataaataatcaggaagaattggttggccttatgtgccaatgaatactcttggttctgacccttttttggtgggagggtcctccagcaggtgcagcttgcaatgtgtacggggactggatgctatgaaagatgtaatgagagggctcatgagcagagctgcctatccctgggggttcactaacgcctacaggacatcctggcccaagtctgcctgcacaactaaaggcacacttctggtctttaggtccttcgctgtatgagcaagcaaaacctggagaatttcacttgcagaaaatccaccagttgctgcaatagttttatcatagtactacatttgaaaaaaaaatatttaaatagtaaaggagggagccatccaaatgaacaggaactgtggaaaggcagcaataactttatcagaagaatctattaccatctcagagtacaagcacatgcgcagacttttgtaatcaaagatgaaaattcttcaatttgtgtactgctaattttgttaagaaatataagccagccaatatgcttactttgaggccaaaggagcaaggtagtatgaggatgttaagacaccaagtactaaggatattaaggtaaactggtatgcagctgctagagggttcagttttgaaataaagcttagtcttatatccagacaggaagaggcagcacatgctaactttagcacgaaggacaagggtcttctcaaagagacagcctgctctttctcttcttgctctgagataaagtgccaaatagcagctttcaagttctagtgagagaaataaaaataaagctgggctactgcacatcaccaaacaaataggtattttcatatcgcatattacaaagtagaggttgagtatcccttatcagaaatgtttcggaccagaagtgttttggatttcagatgtttttgaaatttggaatatttgaaaaatacaaactggttgaacatcccaaatatgaaatccaaaatgctcaaatgagcatttcctttgagcatcatgtcggtattcaaaaagttttggattttggagcacttgattccaggagctcagcctgtatttagaaattaagcataacttctaaatagagctagctaatacttgctggttgcacttaagtatcatagtaattatcagcataaagtaaaaataagtatttactgcctaaaatgttgaaccaatgttttctgggaccatttctctaaatacacaaatggggagacatactagaaaaccttacaattaaatatgctggtagtgttagggttttagagcaaaacagaaatccaacccccaagaaagtcagggaaaagaagacaaaaatcagaagatgaacagctgcatatttctccacctaacactaggaggaaaaagtagaatatttgaaatacgatatggaatacaaatctgtgccatttagaacataatggtaggacgtagtaaacaagctacatcagcacaggacatggtttattgtcaaccatttaaacatataaacaaaactaagagtaagaaaataaaagacagatgctgtagcaaaagggcatttctctccaacatgattggccattattctccaaaatgtatggttaacagaaaattgaagaaaagtttgtatagagttattttaaatgattgatattttctggtttttttttttttttttttttttttttttgagacagggtcttgctctgtaatccaggctagagtgcaatggcatgatcacagctcattgcagccccaaacccccaggctcaaagtgatcctcctgcttcagcctcccgagtagctgggattaccaagcatgagccaccataccgagcaaatttaaaaaatttttttgtagagacagggtctctctatgttgctcaggctggttttgaactcctggactcaagcaatcctccctgcttcagcctcccaaagtgctgggattacaggcctccatgagcaaccacgcccagctcaagaatgattcacattttaattttcttttgaacaggtttaccactttgtatttgtgttttaggttttaagactaaatctgtgcaataatattccctagggattaaaagtaggggaaatacaaccctctccaaaagcagaaacaaaacttggggtggaaagaggaggtaaaaattacattcgcttttccaaatgagtctgaatcgtaaaaccataaagaatggttttactcattctttgtcagccatttgaaatcaataaactatgattcctacattttgtttgtattacacaaaaagtaaacaacaatgaaagctgtttttaaaagaataaaaaccaccaaccacaaatagaagagaaccccagacggttctcttggagggatgtttatcaccagtgccaaaagcctcccccctctgaaatgtttctctcagttgacaactttcaaatgatttaaagaacatgaagaacaagtagaacatgaagcttggatctgaatagtaaagaataatattggagtggtatttacaaaggagaggcagatatatgtgcctagcaccagatttttcaagtaagcaagttcagccccaaactaactgaagttttacatttttaaactctctccattatttcccagagttggaagctgtgaaatgtttcagcatggtgctattcactaatggtgtgaactcaaaaggtgggttttctgcagctgaactgattctaagtctcaggactccaagatacctccagtccaagtgtcgtggactctactggctttatacacctaatttgggactatccattttttccttctttaaagctggctagggaattccttcactaatgataatgtgtgcaaacacacacacatattgaaaatctataactaattctagcagccaaaagatgtttttccttaccagaaattacccaaagaaagttacattagaaataatatgactaaaaatatatttttaaagctatttaatactcatgatgtctaaactttcaatttattgtctgatttctggatatttctgtattttagattctacagacttcagattctgaagcttgttgaaaaagctaagttcctcaatatggatgaaaatctatctggctgtacttttagaggggaatttttctacttttgaaaaaaattctgaatatttatatatagtattaacagaataccccagtaagtcatatttcagataaatattctatagtataatttgcatcatacccaatattttagatattaaaataagggtaaaatttggaatataatcacttgtctgcatatttcccaatgtaagttttcatgtagaatattaaaatttaaattgatatttggatttataagctgttttccctgtatactatacgtatctattagcaatagagacaattttggagtcatggtatagtgaacctctctggctctccttgcacaaggctccatgagtcagtctgggcagtgcacgctacccttgcataactcactccccacactcaggcttaggggtactaacatgcaatcctaggacaacacttgacactagcactgacattttaaaattcattctcccaagtaataaaaaatatatatatagatagatatacacagagagatctgcagctgtactaattacttcaaatagcagcagacaaggaaaatacacgcttgcttgcttaagtttaaattcattttaagtttgctatattaaatttaaaaattaaaaaaatatcaacttactataaacaatttaaaatatgtataatacaacttcatggtcaaaacatttgaatagtctatgaaaacaggaaatacgttcatctgacatttctgtttagattccattcatgatttttcaatctgtctcttccaaaagaaaccataaagcagttgtcatattttatggcaactaattttgtttagggatttcctcatcacaaaaatactttatttcctattacaggggagttaaagaagaagaaaaaagaaatgagaaacaaagtggctttctccccacttgtcactattctcttcttcaaacattctgtacataagctgtctgagtcttttgaaccatttacaaattgtattttcaaaaattgaagaaaaaatatttagagtctaaaagtgttattttatacactgactatacaatatacattgaatgtttacacatacaaatacatcttaaagataaggttctccaaaggtttttcgacattccatcacccctgtacttggtggtctatcacagttgtgtgtactcttgacttgactaggtgtgagacgatcgtatgccatcttgtactctttatcaaaagcatctatatcaatgttttctcttcccagtgccacaagtgagagaaatagtatttctctgtataaactcctctgtcttttaaaatgtggacacttattcagtgtctctaaaatctgactcattggtccatagacatcattcattttaatgctttttaccatacttttcaacagttcctggttaaatgagttatcacttttttgcaataaatggaccattggatatttttgggctgtaaacgaacaaaagaacagatgaaggaaaatgttctgtgtagaaaggagaaagaaattaagcagcaactgacagatattaagttacaaagcactaaaaataaattaagggcaatagataaagaaataggaatccaagaatgaagaaagcaaaaaataagacaaataatgacaaaaaaaggtctaaagctttctgtggtcttaaatagacaataactaagaatattgtttcccttaatacagcctctgatgaaaattctaaatcagcagcctgggatggaaacaaataaaaaataagtaaaaagaagaaattgggatgagcaatgtgctgaaagctgaattctgcaaaacacaaccaacccctccagcacatacacagcacccctcaaaaaaccaaaccaaaacaaaaaacaaaaaacaaaaaaaaacccttagacctccatagaaggtagcactaaaaaaatcaaacactcactctcaaacaaaagagtacgactttgacctgtaagacaaaaagtagtacagtaaaataaaagtcagttatacattggtttatgctatttaaagctagtagagattactctcatatgaacaaagtcagcattctatgatggcacttactgtgtgcattccagagaatgtacaagggctgtcccggatcctgatgtaacttcatattgtcccataacatttgtattaaaacatatttgctatcttcagacatacagtggcggggaatctgtgttatacaataaacattcattaatgatccttacatgataatttttcataagtattttataaaattcttataaatattttttaggatgtatatgtgcgagacagaaaagagaacagaaaaagactgatttatctacatttgatatctactacaggaagatgggctgtgtggaaaagctaatgatctctaaagatcagatataacaaagtacttgagatccgtgagaaagggtaccaagaagaactcatcttgctcctcttgctcatgattgaaagtcacagaaagataaatccaggagtcccatcctatatcatccaacaccctggcccagataacgctgagttcacatctttgtcactcatgtatgatgtactgaaaatccgaagcacatgcacaatcataggcatgcagcacaagaagagagaaggcaaggttcctgaacttagagaccaccatttagtggcagtggcagtatatgaaaaagtaaagacacttttataaaacaacataccgaaaatacaaatgaacatataacaaacaaatggcctaaatgttaaacaaaaatccagggtaaaggaatgacgagagtggtagcacatgattgcaatatgaatttcaatagtccccctttatcctcagcagctatattccaagacctccaatggatacctataactgcagatagtaccgaaccctatatatactgtattttcctatacatacatacttgtgatatttaatttataaatgaggcacaaaaagaaattaacaataactaataataaaatagaacaattaaaacaatatgccagcatcactgctttgtgccattaagtaaaacaggagttacatgaacacaagcactgtgataccatcacagtgggtctgataacagagatggctactcaatgattaacaagcaggtggcatacacagcgtggatacaccgaacaaagggatgattcacatcccagatgggacagcacgaaatttcatcatgctactcagaacagcatgcaatttaaaacttatgaagtgtttctttctggaagtttccacttaatattttgagaccacagttaccatgggtaactgaaacctcagaaaggaaaaccatgaataaggagggactgctgtatagatatccttaaaaagtgttaggcttgggctggacacagtggctcctgcctataaccccagcactttgggaggctgagacaggagggtcacttgagcccaggggttagaggtcacagtgagccatgaccacaccactgcactccagtctgggtgacagggcgagaccttgtgtcaaaaaaaaaaaaaaaaaaaaattaggcttgttttgaaagaagtacaagatgtaagtgggcctaactcacaaatctgcttcctaagagtcatttccagtttattcttgaagcaatagcaaaaattcaagtacgtttaatgtaaattttaggagaaggcaaaaaaaaaagactcttattgctagcctgtaagaagaaaatattatttgtaaatacaactaaaacaattctatttatctaatgacccagagggctattaaaaatatttagcataggctgggcacggtggctcacgcctgtaatcccaacactttgggaggctgaggcaggtggatcataaggtcaagaaatcaagaccatcctggccaacatggtgaaaccccgtctctactaaaaatacaaaaattagctgagcgtggtggtgtgtgcctgcaatcccagctacttgggaggctgaggcaggagaattgcttgaaccctgtagctggaggctgcagtgagccgagatagtgccactgcactccagcctggcgaaagagtgagactacgtctcaaaaaataaaataaaataaatttagcataaaaacagaccttactttttaatcattaggaatatgcaaacattacaatggtaacagaagcattcattgccttttaatttttagtctcatacctttgaatacttgttacagtgctcagaagaaagaatcaatccaggtaagttactgggcaagtcaagacgtctgaaataccataccaggttccaaaaaacaattggatgatggtccacaaagtctgctactgttattgcatgatcaccttcattttccaataagctttcaagttctttccataccactaaaggactaagatacggaacagtgacaggatcgggacttggaaggtgccattctaaacctaaagaatctgtagctccttgtaaagtagctggcaggctgcctgtagaaatgagcttctgtcttccagtatcttccttatccaaggggccagaagtactaatactcctggccattggaaatattggacatttagacatagctgtttttgatctattagcagggatctgaatacttcgggtgcaaaaattttcctgcagtttagatttgctatttagatcaaaattcccttgaacagagagagcagatgtgtcaagaccagaggctgatgttgaaatgcaagactgcctcgtctgacttgaaatggaggatggaaagtgcatattttctgttgatgggcttgactttagaaagtatcttccaggtcgtcttaaatctcttatttctatattcagaaagggtaagaagatattgccacagaatgggcatgtagtattgagatttgaatcatctgctgtccagccagccatgatttcctcatcatggacaagacaatcacaagttctacaccgagagcaacttgagatgagaacctccattgcatagttctggaagatatttgtattactcgcgttgaaggaagatgtcacttctgatttcccaggtaaggcaaacttcgacagagatccttccaaggatgcagaactttccaggcttattcggctgagatcaattctcttagtccctgaagtagcactggtctcttgagaggagataggtccttccaactcatggcagacatcttcatctgttaaagaggtagattcagaatcctgggctcccactgaagaaagactggtacgatcagaactttgatccttagatgatgtggtgtacatggtgaatcttgaataccatttgcttgctttctctgcaactccttttccagcagtgaacatactgtttcttagaacatctagtttaggtactagtagtgtatctaagttaaatgaaggtgatgagtgggttaatgtatcctgagattcttccctaaatgggcaagtaggtgagaaggctggagaagaccaaagtctatcccttggtttctcctcactttttgtgtaacttttagatttggtaagtctcactggcttaggagaattaggaggcagactagatcttctgcatgccttgaccaatggtggacttttcttatttaatttatcatcacatgcccgttgtaaatcaatgcttggtgtacgacttgtcaaaggactgctcatgttattcatatacatcacaatttcttcagctaaatcacgcctagcagatggtgttgaaatgcttttgctatcatcttcatcctcctcctcttcttctttttgctgctgttcagtctcagcaaccaaaagagagaggggatcaaatcctgttgcgacatcagttttttcaaaaggttttactgaaaagctgctgttcatacgttgaatcctcttgggattttgtgtagcaacacatcctgcttttgatacatctgtttcactgtctaagtcttctaagtcaaaaataacaggagaatccactttatctgccaaatagttagaaccatcaaaaggtgtatcatcatcactagattccttttctagactgtctctttttgatcttaaaggtggcttcccaatatcaagagtatttggtctcgtgctttttgagataacatttgaaagaatttttgcatcagctcccaatttttcaactatatctccaggggttgcttcctggttaattctattgagcataaatcccatcagtacccctccactaagattacggtttctatttccccagaccacttgctgctgcaaattagtttcattgtcacttttatgtcttttcctgaagcatctactttgaatgtttcgtgtttcatttgtatcttcaagagatgatattaagagcagctcaggtgtgctttccatgctttctcctgatattttaccagcactgttgttacttgtaccagtgaggcgaacgatactggaagaattttgataactgagcttaggaaggcaatcagcacttccttttgtactctcactctctgacaaggaactacaatcactcccttttttatctttttcttcttgaatgtcttcagtagatgtatcccctcttctaacttcatctttagataatgaattatatccaagatcagactggccacctgtactagatctatcatcagtagcatatactttgattaaacccgtattaaaaggtgcctgctccacagtgtgtgtcccatgaccactatccatgctgccatgactaacagcatccaggtcactgccatctgagagagttgtttgtgataagtgtgcatgcttctttaaagctcttttgaactgtgttactcctaaaacaacatttcttacttttgtccaaagaaaatagccactacgacttcttgaaggccaggtactttccaaaacagccttattataataaccataagtaatggcattggggtcaataccagctttctgcatttcaaaaagcactcgaactgcaagcactggctgatcatattgtccacagagttgcataagaatgcggtagcatacctcatcaggtggatccatcttctttgactgcatttttttaagcacatcatatgctgttttcagagccctgacttttgaatgacagactttcacataagctgggagacaaataaaccacagtccataacagtggcgcagtagacacctagaccacatctgagggatggaagagtacctctttgcaattttatgggctgatttaatttcctgttttgttcttctgaacatgggcaaagggctattaggactacttgattttgaaggcaatttgttcttctttgcttgtagaaatccttcaggtctttcaaataaattgttcctaagaactggaaatccattatagctgtactgtaaagggggttcttcaccattgggtaggtgggggatctcaggtggtgttacaaaaacagtgtgttcacttttgaaagattcatccagttctataagtcgtacttcaccgctcttgtccatatccactttatctacacaatcatcaaaaaatgccaggcttgcatctttgtcactaacaaaagaacattcttcaatgaagcgaataaacatttgtgttttggtcatcatgttatagaatttttgatgtgaccggtcccggcttcttaagaaagcttgtagggcaaagagagaggctgcatctgtggctgtctcagatggggcttgtgttattggccttaagtatgatctgtaaccttttaaaatagaggccatgaaaaacaaaaatgcctcttggatttccaaatctatcatgtgcaacctctttccagaattaaaatcatagtcatttattgctaaatccatgagtccatcatctctcggtctctgctgcaattttgccaattgctgatgcaaattattcagtgtgttcatcagatttttacatggcttctttggaagtatcttccaggctacatttttcttgtcaccaatttgagaaatagtgttggtatctacatcaacacaactgacatctggtggaggatcatagagatcaaagtatcttgaatcaatccctactatgaatggacatggtgcactcaagacatctgctaaagccagtgggcagagaggaacatacgggcatggccagtggaaagggaaaatcatagacactaatgcttctgtcacactagtaagcacggatggccgtagggaatggataagaattttatgttctgttactgcaaacaccagtagtgtcacagcattttcagggcctaaattctgcagtagtgttgaaaacttgccaccacttagtggaagaggtgaagacacaggctgactgagaatcagattatcatgtggtgataactgaactaaaatccgtggtctctgaggagatggaaaaggaactttatgcataaaatgagaaatatgcttctcaattggaaggacatgaggcccagagatggaataacgatacagaaaagtcagaaacttcctgaatgcatcaaaaaaaggccagtgagaaagaagacagatgcatttgttagtatgaattgttttggaactatcagacttcccatctgctgatgttaaacccaaaagaagtctctgcttttctgtgagattctcctcagagtatggttcataaaactgaatagcagcaccataaaccttttcagctgaggctccagttaaaacaaaagtagaaaatacaggcagagggtatttgctatttgatggccaacattcaatggttgcacccattggtaaacaaaatagaggaacagattccggtagtgagaatgactcataatcttcttgaggatatctacaaattaggccagctttgtaagatacagtgttcgtctttgccaccgattttttataacacaagtatactgctgatccccacatactgttattgagattcttgtcgactttgcagaacgtgtgtggtgggctttctcctttactgggtataataatacatatgtcagtgacagccaacgtattctgagtcatgttttcagaggctcttcggtaagtgatataaattctttgtgatgaggtactcccactaatatttgcggggcgcccatagggagtactctgaataatttcacaaccctgtttcaatctttctttccagtcatataaaacccccagatctgtaagtggaggcttatctcttcctcttctatagcaaaggtaaatctgtggccccacaagacttccattattaagatcagctgacaatccagttggggtaacatcaatacagatataatcctgtgggacttcctccccaagagatttgataataactgaaacatctgtaataggttcttttggtttagctactttatgacaagcatcattgaagtgaatttcttcttctagaggctttgaaacatcagttaatcctgctacaacaaagtagtcagcaacacgaggccccttgtcttcaatcatcttccattacagaaggttacatacattaccgaaagtttctctctgaaaaagatgacagatttcaatgtgtgaactccgcagcctcagagtttgagaaataactctccgggccgtgacagctccacctgccaccgctgcccgggtcgccgcccccgcactcaccacccagctggctcccgtgcgagcagcggatcgagctcggagagcggcgccggaatcccgcacgcgcggtagcggaacacgaggggctgaatgccgcggcgctctgagcccgcttagctcatccccagcccggcgctccgc

SEQ ID NO: 15509 - RNA, 10864 nt, Homo sapiens
  source 1..10864: mol_type = other RNA
gctgggattacaggcatgagccactgtacccagccaaaatggttactatatattttgaacattatattgcactgtcatcaatagattcgaaaatagttttaccaaattacaggcttagtcttttatagctgtctatatcaatattatttaaagattgagtaccaaagggggcaggaattggaatgtattatctagagcacagaatagtaaataatcaggaaaagggccgggcgcggtggctcatgcctataatcccagcactttgggaggccaaggtgggcggatcacgaggtcagtagatcgagaccatcctggctaacacggtgaaaccccgtctctactaaaaaaataccaaaaattagccgggcgaggtggcaggcgcctatagtcccagctactcgggaggctgaggcaggagaatggcgtgaaccccggggggcggagcctgcagtgagccgagatcgtgccactgcactccagcctgggcaacagcgagactccgtctcaaaaaaaaagaaaaaataaataatcaggaagaattggttggccttatgtgccaatgaatactcttggttctgacccttttttggtgggagggtcctccagcaggtgcagcttgcaatgtgtacggggactggatgctatgaaagatgtaatgagagggctcatgagcagagctgcctatccctgggggttcactaacgcctacaggacatcctggcccaagtctgcctgcacaactaaaggcacacttctggtctttaggtccttcgctgtatgagcaagcaaaacctggagaatttcacttgcagaaaatccaccagttgctgcaatagttttatcatagtactacatttgaaaaaaaaatatttaaatagtaaaggagggagccatccaaatgaacaggaactgtggaaaggcagcaataactttatcagaagaatctattaccatctcagagtacaagcacatgcgcagacttttgtaatcaaagatgaaaattcttcaatttgtgtactgctaattttgttaagaaatataagccagccaatatgcttactttgaggccaaaggagcaaggtagtatgaggatgttaagacaccaagtactaaggatattaaggtaaactggtatgcagctgctagagggttcagttttgaaataaagcttagtcttatatccagacaggaagaggcagcacatgctaactttagcacgaaggacaagggtcttctcaaagagacagcctgctctttctcttcttgctctgagataaagtgccaaatagcagctttcaagttctagtgagagaaataaaaataaagctgggctactgcacatcaccaaacaaataggtattttcatatcgcatattacaaagtagaggttgagtatcccttatcagaaatgtttcggaccagaagtgttttggatttcagatgtttttgaaatttggaatatttgaaaaatacaaactggttgaacatcccaaatatgaaatccaaaatgctcaaatgagcatttcctttgagcatcatgtcggtattcaaaaagttttggattttggagcacttgattccaggagctcagcctgtatttagaaattaagcataacttctaaatagagctagctaatacttgctggttgcacttaagtatcatagtaattatcagcataaagtaaaaataagtatttactgcctaaaatgttgaaccaatgttttctgggaccatttctctaaatacacaaatggggagacatactagaaaaccttacaattaaatatgctggtagtgttagggttttagagcaaaacagaaatccaacccccaagaaagtcagggaaaagaagacaaaaatcagaagatgaacagctgcatatttctccacctaacactaggaggaaaaagtagaatatttgaaatacgatatggaatacaaatctgtgccatttagaacataatggtaggacgtagtaaacaagctacatcagcacaggacatggtttattgtcaaccatttaaacatataaacaaaactaagagtaagaaaataaaagacagatgctgtagcaaaagggcatttctctccaacatgattggccattattctccaaaatgtatggttaacagaaaattgaagaaaagtttgtatagagttattttaaatgattgatattttctggtttttttttttttttttttttttttttttgagacagggtcttgctctgtaatccaggctagagtgcaatggcatgatcacagctcattgcagccccaaacccccaggctcaaagtgatcctcctgcttcagcctcccgagtagctgggattaccaagcatgagccaccataccgagcaaatttaaaaaatttttttgtagagacagggtctctctatgttgctcaggctggttttgaactcctggactcaagcaatcctccctgcttcagcctcccaaagtgctgggattacaggcctccatgagcaaccacgcccagctcaagaatgattcacattttaattttcttttgaacaggtttaccactttgtatttgtgttttaggttttaagactaaatctgtgcaataatattccctagggattaaaagtaggggaaatacaaccctctccaaaagcagaaacaaaacttggggtggaaagaggaggtaaaaattacattcgcttttccaaatgagtctgaatcgtaaaaccataaagaatggttttactcattctttgtcagccatttgaaatcaataaactatgattcctacattttgtttgtattacacaaaaagtaaacaacaatgaaagctgtttttaaaagaataaaaaccaccaaccacaaatagaagagaaccccagacggttctcttggagggatgtttatcaccagtgccaaaagcctcccccctctgaaatgtttctctcagttgacaactttcaaatgatttaaagaacatgaagaacaagtagaacatgaagcttggatctgaatagtaaagaataatattggagtggtatttacaaaggagaggcagatatatgtgcctagcaccagatttttcaagtaagcaagttcagccccaaactaactgaagttttacatttttaaactctctccattatttcccagagttggaagctgtgaaatgtttcagcatggtgctattcactaatggtgtgaactcaaaaggtgggttttctgcagctgaactgattctaagtctcaggactccaagatacctccagtccaagtgtcgtggactctactggctttatacacctaatttgggactatccattttttccttctttaaagctggctagggaattccttcactaatgataatgtgtgcaaacacacacacatattgaaaatctataactaattctagcagccaaaagatgtttttccttaccagaaattacccaaagaaagttacattagaaataatatgactaaaaatatatttttaaagctatttaatactcatgatgtctaaactttcaatttattgtctgatttctggatatttctgtattttagattctacagacttcagattctgaagcttgttgaaaaagctaagttcctcaatatggatgaaaatctatctggctgtacttttagaggggaatttttctacttttgaaaaaaattctgaatatttatatatagtattaacagaataccccagtaagtcatatttcagataaatattctatagtataatttgcatcatacccaatattttagatattaaaataagggtaaaatttggaatataatcacttgtctgcatatttcccaatgtaagttttcatgtagaatattaaaatttaaattgatatttggatttataagctgttttccctgtatactatacgtatctattagcaatagagacaattttggagtcatggtatagtgaacctctctggctctccttgcacaaggctccatgagtcagtctgggcagtgcacgctacccttgcataactcactccccacactcaggcttaggggtactaacatgcaatcctaggacaacacttgacactagcactgacattttaaaattcattctcccaagtaataaaaaatatatatatagatagatatacacagagagatctgcagctgtactaattacttcaaatagcagcagacaaggaaaatacacgcttgcttgcttaagtttaaattcattttaagtttgctatattaaatttaaaaattaaaaaaatatcaacttactataaacaatttaaaatatgtataatacaacttcatggtcaaaacatttgaatagtctatgaaaacaggaaatacgttcatctgacatttctgtttagattccattcatgatttttcaatctgtctcttccaaaagaaaccataaagcagttgtcatattttatggcaactaattttgtttagggatttcctcatcacaaaaatactttatttcctattacaggggagttaaagaagaagaaaaaagaaatgagaaacaaagtggctttctccccacttgtcactattctcttcttcaaacattctgtacataagctgtctgagtcttttgaaccatttacaaattgtattttcaaaaattgaagaaaaaatatttagagtctaaaagtgttattttatacactgactatacaatatacattgaatgtttacacatacaaatacatcttaaagataaggttctccaaaggtttttcgacattccatcacccctgtacttggtggtctatcacagttgtgtgtactcttgacttgactaggtgtgagacgatcgtatgccatcttgtactctttatcaaaagcatctatatcaatgttttctcttcccagtgccacaagtgagagaaatagtatttctctgtataaactcctctgtcttttaaaatgtggacacttattcagtgtctctaaaatctgactcattggtccatagacatcattcattttaatgctttttaccatacttttcaacagttcctggttaaatgagttatcacttttttgcaataaatggaccattggatatttttgggtgtgtgcattccagagaatgtacaagggctgtcccggatcctgatgtaacttcatattgtcccataacatttgtattaaaacatatttgctatcttcagacatacagtggcggggaatctttgaatacttgttacagtgctcagaagaaagaatcaatccaggtaagttactgggcaagtcaagacgtctgaaataccataccaggttccaaaaaacaattggatgatggtccacaaagtctgctactgttattgcatgatcaccttcattttccaataagctttcaagttctttccataccactaaaggactaagatacggaacagtgacaggatcgggacttggaaggtgccattctaaacctaaagaatctgtagctccttgtaaagtagctggcaggctgcctgtagaaatgagcttctgtcttccagtatcttccttatccaaggggccagaagtactaatactcctggccattggaaatattggacatttagacatagctgtttttgatctattagcagggatctgaatacttcgggtgcaaaaattttcctgcagtttagatttgctatttagatcaaaattcccttgaacagagagagcagatgtgtcaagaccagaggctgatgttgaaatgcaagactgcctcgtctgacttgaaatggaggatggaaagtgcatattttctgttgatgggcttgactttagaaagtatcttccaggtcgtcttaaatctcttatttctatattcagaaagggtaagaagatattgccacagaatgggcatgtagtattgagatttgaatcatctgctgtccagccagccatgatttcctcatcatggacaagacaatcacaagttctacaccgagagcaacttgagatgagaacctccattgcatagttctggaagatatttgtattactcgcgttgaaggaagatgtcacttctgatttcccaggtaaggcaaacttcgacagagatccttccaaggatgcagaactttccaggcttattcggctgagatcaattctcttagtccctgaagtagcactggtctcttgagaggagataggtccttccaactcatggcagacatcttcatctgttaaagaggtagattcagaatcctgggctcccactgaagaaagactggtacgatcagaactttgatcctgggcttcattcacaagaacagttctcatcttggtagctgatctctcttatgactactttggaggctatactttctgtattcaggcattttcatcaatccagtttcatttgctttctcattttcagaaaggtatgaaaatttctcatctcctgatggcatacttttcttctttcattgctttgatggatttattatattctcctatttttctgtcacttagatgatgtggtgtacatggtgaatcttgaataccatttgcttgctttctctgcaactccttttccagcagtgaacatactgtttcttagaacatctagtttaggtactagtagtgtatctaagttaaatgaaggtgatgagtgggttaatgtatcctgagattcttccctaaatgggcaagtaggtgagaaggctggagaagaccaaagtctatcccttggtttctcctcactttttgtgtaacttttagatttggtaagtctcactggcttaggagaattaggaggcagactagatcttctgcatgccttgaccaatggtggacttttcttatttaatttatcatcacatgcccgttgtaaatcaatgcttggtgtacgacttgtcaaaggactgctcatgttattcatatacatcacaatttcttcagctaaatcacgcctagcagatggtgttgaaatgcttttgctatcatcttcatcctcctcctcttcttctttttgctgctgttcagtctcagcaaccaaaagagagaggggatcaaatcctgttgcgacatcagttttttcaaaaggttttactgaaaagctgctgttcatacgttgaatcctcttgggattttgtgtagcaacacatcctgcttttgatacatctgtttcactgtctaagtcttctaagtcaaaaataacaggagaatccactttatctgccaaatagttagaaccatcaaaaggtgtatcatcatcactagattccttttctagactgtctctttttgatcttaaaggtggcttcccaatatcaagagtatttggtctcgtgctttttgagataacatttgaaagaatttttgcatcagctcccaatttttcaactatatctccaggggttgcttcctggttaattctattgagcataaatcccatcagtacccctccactaagattacggtttctatttccccagaccacttgctgctgcaaattagtttcattgtcacttttatgtcttttcctgaagcatctactttgaatgtttcgtgtttcatttgtatcttcaagagatgatattaagagcagctcaggtgtgctttccatgctttctcctgatattttaccagcactgttgttacttgtaccagtgaggcgaacgatactggaagaattttgataactgagcttaggaaggcaatcagcacttccttttgtactctcactctctgacaaggaactacaatcactcccttttttatctttttcttcttgaatgtcttcagtagatgtatcccctcttctaacttcatctttagataatgaattatatccaagatcagactggccacctgagagagttgtttgtgataagtgtgcatgcttctttaaagctcttttgaactgtgttactcctaaaacaacatttcttacttttgtccaaagaaaatagccactacgacttcttgaaggccaggtactttccaaaacagccttattataataaccataagtaatggcattggggtcaataccagctttctgcatttcaaaaagcactcgaactgcaagcactggctgatcatattgtccacagagttgcataagaatgcggtagcatacctcatcaggtggatccatcttctttgactgcatttttttaagcacatcatatgctgttttcagagccctgacttttgaatgacagactttcacataagctgggagacaaataaaccacagtccataacagtggcgcagtagacacctagaccacatctgagggatggaagagtacctctttgcaattttatgggctgatttaatttcctgttttgttcttctgaacatgggcaaagggctattaggactacttgattttgaaggcaatttgttcttctttgcttgtagaaatccttcaggtctttcaaataaattgttcctaagaactggaaatccattatagctgtactgtaaagggggttcttcaccattgggtaggtgggggatctcaggtggtgttacaaaaacagtgtgttcacttttgaaagattcatccagttctataagtcgtacttcaccgctcttgtccatatccactttatctacacaatcatcaaaaaatgccaggcttgcatctttgtcactaacaaaagaacattcttcaatgaagcgaataaacatttgtgttttggtcatcatgttatagaatttttgatgtgaccggtcccggcttcttaagaaagcttgtagggcaaagagagaggctgcatctgtggctgtctcagatggggcttgtgttattggccttaagtatgatctgtaaccttttaaaatagaggccatgaaaaacaaaaatgcctcttggatttccaaatctatcatgtgcaacctctttccagaattaaaatcatagtcatttattgctaaatccatgagtccatcatctctcggtctctgctgcaattttgccaattgctgatgcaaattattcagtgtgttcatcagatttttacatggcttctttggaagtatcttccaggctacatttttcttgtcaccaatttgagaaatagtgttggtatctacatcaacacaactgacatctggtggaggatcatagagatcaaagtatcttgaatcaatccctactatgaatggacatggtgcactcaagacatctgctaaagccagtgggcagagaggaacatacgggcatggccagtggaaagggaaaatcatagacactaatgcttctgtcacactagtaagcacggatggccgtagggaatggataagaattttatgttctgttactgcaaacaccagtagtgtcacagcattttcagggcctaaattctgcagtagtgttgaaaacttgccaccacttagtggaagaggtgaagacacaggctgactgagaatcagattatcatgtggtgataactgaactaaaatccgtggtctctgaggagatggaaaaggaactttatgcataaaatgagaaatatgcttctcaattggaaggacatgaggcccagagatggaataacgatacagaaaagtcagaaacttcctgaatgcatcaaaaaaaggccagtgagaaagaagacagatgcatttgttagtatgaattgttttggaactatcagacttcccatctgctgatgttaaacccaaaagaagtctctgcttttctgtgagattctcctcagagtatggttcataaaactgaatagcagcaccataaaccttttcagctgaggctccagttaaaacaaaagtagaaaatacaggcagagggtatttgctatttgatggccaacattcaatggttgcacccattggtaaacaaaatagaggaacagattccggtagtgagaatgactcataatcttcttgaggatatctacaaattaggccagctttgtaagatacagtgttcgtctttgccaccgattttttataacacaagtatactgctgatccccacatactgttattgagattcttgtcgactttgcagaacgtgtgtggtgggctttctcctttactgggtataataatacatatgtcagtgacagccaacgtattctgagtcatgttttcagaggctcttcggtaagtgatataaattctttgtgatgaggtactcccactaatatttgcggggcgcccatagggagtactctgaataatttcacaaccctgtttcaatctttctttccagtcatataaaacccccagatctgtaagtggaggcttatctcttcctcttctatagcaaaggtaaatctgtggccccacaagacttccattattaagatcagctgacaatccagttggggtaacatcaatacagatataatcctgtgggacttcctccccaagagatttgataataactgaaacatctgtaataggttcttttggtttagctactttatgacaagcatcattgaagtgaatttcttcttctagaggctttgaaacatcagttaatcctgctacaacaaagtagtcagcaacacgaggccccttgtcttcaatcatcttccattacagaaggttacatacattaccgaaagtttctctctgaaaaagatgacagatttcaatgtgtgaactccgcagcctcagagtttgagaaataacacccagctggctcccgtgcgagcagcggatcgagctcggagagcggcgccggaatcccgcacgcgcggtagcggaacacgaggggctgaatgccgcggcgctctgagcccgcttagctcatccccagcccggcgctccgcccttcgcggcacccccgcccgcccgcccaggcctgccgtctcagtcagacgggactccccctcccctcgcggccgccactgcctccgcctctttctcc

SEQ ID NO: 15510 - RNA, 10623 nt, Homo sapiens
  source 1..10623: mol_type = other RNA
gctgggattacaggcatgagccactgtacccagccaaaatggttactatatattttgaacattatattgcactgtcatcaatagattcgaaaatagttttaccaaattacaggcttagtcttttatagctgtctatatcaatattatttaaagattgagtaccaaagggggcaggaattggaatgtattatctagagcacagaatagtaaataatcaggaaaagggccgggcgcggtggctcatgcctataatcccagcactttgggaggccaaggtgggcggatcacgaggtcagtagatcgagaccatcctggctaacacggtgaaaccccgtctctactaaaaaaataccaaaaattagccgggcgaggtggcaggcgcctatagtcccagctactcgggaggctgaggcaggagaatggcgtgaaccccggggggcggagcctgcagtgagccgagatcgtgccactgcactccagcctgggcaacagcgagactccgtctcaaaaaaaaagaaaaaataaataatcaggaagaattggttggccttatgtgccaatgaatactcttggttctgacccttttttggtgggagggtcctccagcaggtgcagcttgcaatgtgtacggggactggatgctatgaaagatgtaatgagagggctcatgagcagagctgcctatccctgggggttcactaacgcctacaggacatcctggcccaagtctgcctgcacaactaaaggcacacttctggtctttaggtccttcgctgtatgagcaagcaaaacctggagaatttcacttgcagaaaatccaccagttgctgcaatagttttatcatagtactacatttgaaaaaaaaatatttaaatagtaaaggagggagccatccaaatgaacaggaactgtggaaaggcagcaataactttatcagaagaatctattaccatctcagagtacaagcacatgcgcagacttttgtaatcaaagatgaaaattcttcaatttgtgtactgctaattttgttaagaaatataagccagccaatatgcttactttgaggccaaaggagcaaggtagtatgaggatgttaagacaccaagtactaaggatattaaggtaaactggtatgcagctgctagagggttcagttttgaaataaagcttagtcttatatccagacaggaagaggcagcacatgctaactttagcacgaaggacaagggtcttctcaaagagacagcctgctctttctcttcttgctctgagataaagtgccaaatagcagctttcaagttctagtgagagaaataaaaataaagctgggctactgcacatcaccaaacaaataggtattttcatatcgcatattacaaagtagaggttgagtatcccttatcagaaatgtttcggaccagaagtgttttggatttcagatgtttttgaaatttggaatatttgaaaaatacaaactggttgaacatcccaaatatgaaatccaaaatgctcaaatgagcatttcctttgagcatcatgtcggtattcaaaaagttttggattttggagcacttgattccaggagctcagcctgtatttagaaattaagcataacttctaaatagagctagctaatacttgctggttgcacttaagtatcatagtaattatcagcataaagtaaaaataagtatttactgcctaaaatgttgaaccaatgttttctgggaccatttctctaaatacacaaatggggagacatactagaaaaccttacaattaaatatgctggtagtgttagggttttagagcaaaacagaaatccaacccccaagaaagtcagggaaaagaagacaaaaatcagaagatgaacagctgcatatttctccacctaacactaggaggaaaaagtagaatatttgaaatacgatatggaatacaaatctgtgccatttagaacataatggtaggacgtagtaaacaagctacatcagcacaggacatggtttattgtcaaccatttaaacatataaacaaaactaagagtaagaaaataaaagacagatgctgtagcaaaagggcatttctctccaacatgattggccattattctccaaaatgtatggttaacagaaaattgaagaaaagtttgtatagagttattttaaatgattgatattttctggtttttttttttttttttttttttttttttgagacagggtcttgctctgtaatccaggctagagtgcaatggcatgatcacagctcattgcagccccaaacccccaggctcaaagtgatcctcctgcttcagcctcccgagtagctgggattaccaagcatgagccaccataccgagcaaatttaaaaaatttttttgtagagacagggtctctctatgttgctcaggctggttttgaactcctggactcaagcaatcctccctgcttcagcctcccaaagtgctgggattacaggcctccatgagcaaccacgcccagctcaagaatgattcacattttaattttcttttgaacaggtttaccactttgtatttgtgttttaggttttaagactaaatctgtgcaataatattccctagggattaaaagtaggggaaatacaaccctctccaaaagcagaaacaaaacttggggtggaaagaggaggtaaaaattacattcgcttttccaaatgagtctgaatcgtaaaaccataaagaatggttttactcattctttgtcagccatttgaaatcaataaactatgattcctacattttgtttgtattacacaaaaagtaaacaacaatgaaagctgtttttaaaagaataaaaaccaccaaccacaaatagaagagaaccccagacggttctcttggagggatgtttatcaccagtgccaaaagcctcccccctctgaaatgtttctctcagttgacaactttcaaatgatttaaagaacatgaagaacaagtagaacatgaagcttggatctgaatagtaaagaataatattggagtggtatttacaaaggagaggcagatatatgtgcctagcaccagatttttcaagtaagcaagttcagccccaaactaactgaagttttacatttttaaactctctccattatttcccagagttggaagctgtgaaatgtttcagcatggtgctattcactaatggtgtgaactcaaaaggtgggttttctgcagctgaactgattctaagtctcaggactccaagatacctccagtccaagtgtcgtggactctactggctttatacacctaatttgggactatccattttttccttctttaaagctggctagggaattccttcactaatgataatgtgtgcaaacacacacacatattgaaaatctataactaattctagcagccaaaagatgtttttccttaccagaaattacccaaagaaagttacattagaaataatatgactaaaaatatatttttaaagctatttaatactcatgatgtctaaactttcaatttattgtctgatttctggatatttctgtattttagattctacagacttcagattctgaagcttgttgaaaaagctaagttcctcaatatggatgaaaatctatctggctgtacttttagaggggaatttttctacttttgaaaaaaattctgaatatttatatatagtattaacagaataccccagtaagtcatatttcagataaatattctatagtataatttgcatcatacccaatattttagatattaaaataagggtaaaatttggaatataatcacttgtctgcatatttcccaatgtaagttttcatgtagaatattaaaatttaaattgatatttggatttataagctgttttccctgtatactatacgtatctattagcaatagagacaattttggagtcatggtatagtgaacctctctggctctccttgcacaaggctccatgagtcagtctgggcagtgcacgctacccttgcataactcactccccacactcaggcttaggggtactaacatgcaatcctaggacaacacttgacactagcactgacattttaaaattcattctcccaagtaataaaaaatatatatatagatagatatacacagagagatctgcagctgtactaattacttcaaatagcagcagacaaggaaaatacacgcttgcttgcttaagtttaaattcattttaagtttgctatattaaatttaaaaattaaaaaaatatcaacttactataaacaatttaaaatatgtataatacaacttcatggtcaaaacatttgaatagtctatgaaaacaggaaatacgttcatctgacatttctgtttagattccattcatgatttttcaatctgtctcttccaaaagaaaccataaagcagttgtcatattttatggcaactaattttgtttagggatttcctcatcacaaaaatactttatttcctattacaggggagttaaagaagaagaaaaaagaaatgagaaacaaagtggctttctccccacttgtcactattctcttcttcaaacattctgtacataagctgtctgagtcttttgaaccatttacaaattgtattttcaaaaattgaagaaaaaatatttagagtctaaaagtgttattttatacactgactatacaatatacattgaatgtttacacatacaaatacatcttaaagataaggttctccaaaggtttttcgacattccatcacccctgtacttggtggtctatcacagttgtgtgtactcttgacttgactaggtgtgagacgatcgtatgccatcttgtactctttatcaaaagcatctatatcaatgttttctcttcccagtgccacaagtgagagaaatagtatttctctgtataaactcctctgtcttttaaaatgtggacacttattcagtgtctctaaaatctgactcattggtccatagacatcattcattttaatgctttttaccatacttttcaacagttcctggttaaatgagttatcacttttttgcaataaatggaccattggatatttttgggtgtgtgcattccagagaatgtacaagggctgtcccggatcctgatgtaacttcatattgtcccataacatttgtattaaaacatatttgctatcttcagacatacagtggcggggaatctttgaatacttgttacagtgctcagaagaaagaatcaatccaggtaagttactgggcaagtcaagacgtctgaaataccataccaggttccaaaaaacaattggatgatggtccacaaagtctgctactgttattgcatgatcaccttcattttccaataagctttcaagttctttccataccactaaaggactaagatacggaacagtgacaggatcgggacttggaaggtgccattctaaacctaaagaatctgtagctccttgtaaagtagctggcaggctgcctgtagaaatgagcttctgtcttccagtatcttccttatccaaggggccagaagtactaatactcctggccattggaaatattggacatttagacatagctgtttttgatctattagcagggatctgaatacttcgggtgcaaaaattttcctgcagtttagatttgctatttagatcaaaattcccttgaacagagagagcagatgtgtcaagaccagaggctgatgttgaaatgcaagactgcctcgtctgacttgaaatggaggatggaaagtgcatattttctgttgatgggcttgactttagaaagtatcttccaggtcgtcttaaatctcttatttctatattcagaaagggtaagaagatattgccacagaatgggcatgtagtattgagatttgaatcatctgctgtccagccagccatgatttcctcatcatggacaagacaatcacaagttctacaccgagagcaacttgagatgagaacctccattgcatagttctggaagatatttgtattactcgcgttgaaggaagatgtcacttctgatttcccaggtaaggcaaacttcgacagagatccttccaaggatgcagaactttccaggcttattcggctgagatcaattctcttagtccctgaagtagcactggtctcttgagaggagataggtccttccaactcatggcagacatcttcatctgttaaagaggtagattcagaatcctgggctcccactgaagaaagactggtacgatcagaactttgatccttagatgatgtggtgtacatggtgaatcttgaataccatttgcttgctttctctgcaactccttttccagcagtgaacatactgtttcttagaacatctagtttaggtactagtagtgtatctaagttaaatgaaggtgatgagtgggttaatgtatcctgagattcttccctaaatgggcaagtaggtgagaaggctggagaagaccaaagtctatcccttggtttctcctcactttttgtgtaacttttagatttggtaagtctcactggcttaggagaattaggaggcagactagatcttctgcatgccttgaccaatggtggacttttcttatttaatttatcatcacatgcccgttgtaaatcaatgcttggtgtacgacttgtcaaaggactgctcatgttattcatatacatcacaatttcttcagctaaatcacgcctagcagatggtgttgaaatgcttttgctatcatcttcatcctcctcctcttcttctttttgctgctgttcagtctcagcaaccaaaagagagaggggatcaaatcctgttgcgacatcagttttttcaaaaggttttactgaaaagctgctgttcatacgttgaatcctcttgggattttgtgtagcaacacatcctgcttttgatacatctgtttcactgtctaagtcttctaagtcaaaaataacaggagaatccactttatctgccaaatagttagaaccatcaaaaggtgtatcatcatcactagattccttttctagactgtctctttttgatcttaaaggtggcttcccaatatcaagagtatttggtctcgtgctttttgagataacatttgaaagaatttttgcatcagctcccaatttttcaactatatctccaggggttgcttcctggttaattctattgagcataaatcccatcagtacccctccactaagattacggtttctatttccccagaccacttgctgctgcaaattagtttcattgtcacttttatgtcttttcctgaagcatctactttgaatgtttcgtgtttcatttgtatcttcaagagatgatattaagagcagctcaggtgtgctttccatgctttctcctgatattttaccagcactgttgttacttgtaccagtgaggcgaacgatactggaagaattttgataactgagcttaggaaggcaatcagcacttccttttgtactctcactctctgacaaggaactacaatcactcccttttttatctttttcttcttgaatgtcttcagtagatgtatcccctcttctaacttcatctttagataatgaattatatccaagatcagactggccacctgagagagttgtttgtgataagtgtgcatgcttctttaaagctcttttgaactgtgttactcctaaaacaacatttcttacttttgtccaaagaaaatagccactacgacttcttgaaggccaggtactttccaaaacagccttattataataaccataagtaatggcattggggtcaataccagctttctgcatttcaaaaagcactcgaactgcaagcactggctgatcatattgtccacagagttgcataagaatgcggtagcatacctcatcaggtggatccatcttctttgactgcatttttttaagcacatcatatgctgttttcagagccctgacttttgaatgacagactttcacataagctgggagacaaataaaccacagtccataacagtggcgcagtagacacctagaccacatctgagggatggaagagtacctctttgcaattttatgggctgatttaatttcctgttttgttcttctgaacatgggcaaagggctattaggactacttgattttgaaggcaatttgttcttctttgcttgtagaaatccttcaggtctttcaaataaattgttcctaagaactggaaatccattatagcacctaaaaattagggatctgtaaagtttggatttttgaaaataccacagtccttagaaagctacgtcacagatgatggattgcttctctctttcaatctcaaacattctgcctcttgaatacctgtactgtaaagggggttcttcaccattgggtaggtgggggatctcaggtggtgttacaaaaacagtgtgttcacttttgaaagattcatccagttctataagtcgtacttcaccgctcttgtccatatccactttatctacacaatcatcaaaaaatgccaggcttgcatctttgtcactaacaaaagaacattcttcaatgaagcgaataaacatttgtgttttggtcatcatgttatagaatttttgatgtgaccggtcccggcttcttaagaaagcttgtagggcaaagagagaggctgcatctgtggctgtctcagatggggcttgtgttattggccttaagtatgatctgtaaccttttaaaatagaggccatgaaaaacaaaaatgcctcttggatttccaaatctatcatgtgcaacctctttccagaattaaaatcatagtcatttattgctaaatccatgagtccatcatctctcggtctctgctgcaattttgccaattgctgatgcaaattattcagtgtgttcatcagatttttacatggcttctttggaagtatcttccaggctacatttttcttgtcaccaatttgagaaatagtgttggtatctacatcaacacaactgacatctggtggaggatcatagagatcaaagtatcttgaatcaatccctactatgaatggacatggtgcactcaagacatctgctaaagccagtgggcagagaggaacatacgggcatggccagtggaaagggaaaatcatagacactaatgcttctgtcacactagtaagcacggatggccgtagggaatggataagaattttatgttctgttactgcaaacaccagtagtgtcacagcattttcagggcctaaattctgcagtagtgttgaaaacttgccaccacttagtggaagaggtgaagacacaggctgactgagaatcagattatcatgtggtgataactgaactaaaatccgtggtctctgaggagatggaaaaggaactttatgcataaaatgagaaatatgcttctcaattggaaggacatgaggcccagagatggaataacgatacagaaaagtcagaaacttcctgaatgcatcaaaaaaaggccagtgagaaagaagacagatgcatttgttagtatgaattgttttggaactatcagacttcccatctgctgatgttaaacccaaaagaagtctctgcttttctgtgagattctcctcagagtatggttcataaaactgaatagcagcaccataaaccttttcagctgaggctccagttaaaacaaaagtagaaaatacaggcagagggtatttgctatttgatggccaacattcaatggttgcacccattggtaaacaaaatagaggaacagattccggtagtgagaatgactcataatcttcttgaggatatctacaaattaggccagctttgtaagatacagtgttcgtctttgccaccgattttttataacacaagtatactgctgatccccacatactgttattgagattcttgtcgactttgcagaacgtgtgtggtgggctttctcctttactgggtataataatacatatgtcagtgacagccaacgtattctgagtcatgttttcagaggctcttcggtaagtgatataaattctttgtgatgaggtactcccactaatatttgcggggcgcccatagggagtactctgaataatttcacaaccctgtttcaatctttctttccagtcatataaaacccccagatctgtaagtggaggcttatctcttcctcttctatagcaaaggtaaatctgtggccccacaagacttccattattaagatcagctgacaatccagttggggtaacatcaatacagatataatcctgtgggacttcctccccaagagatttgataataactgaaacatctgtaataggttcttttggtttagctactttatgacaagcatcattgaagtgaatttcttcttctagaggctttgaaacatcagttaatcctgctacaacaaagtagtcagcaacacgaggccccttgtcttcaatcatcttccattacagaaggttacatacattaccgaaagtttctctctgaaaaagatgacagatttcaatgtgtgaactccgcagcctcagagtttgagaaataacacccagctggctcccgtgcgagcagcggatcgagctcggagagcggcgccggaatcccgcacgcgcggtagcggaacacgaggggctgaat

SEQ ID NO: 15511 - RNA, 10752 nt, Homo sapiens
  source 1..10752: mol_type = other RNA
gctgggattacaggcatgagccactgtacccagccaaaatggttactatatattttgaacattatattgcactgtcatcaatagattcgaaaatagttttaccaaattacaggcttagtcttttatagctgtctatatcaatattatttaaagattgagtaccaaagggggcaggaattggaatgtattatctagagcacagaatagtaaataatcaggaaaagggccgggcgcggtggctcatgcctataatcccagcactttgggaggccaaggtgggcggatcacgaggtcagtagatcgagaccatcctggctaacacggtgaaaccccgtctctactaaaaaaataccaaaaattagccgggcgaggtggcaggcgcctatagtcccagctactcgggaggctgaggcaggagaatggcgtgaaccccggggggcggagcctgcagtgagccgagatcgtgccactgcactccagcctgggcaacagcgagactccgtctcaaaaaaaaagaaaaaataaataatcaggaagaattggttggccttatgtgccaatgaatactcttggttctgacccttttttggtgggagggtcctccagcaggtgcagcttgcaatgtgtacggggactggatgctatgaaagatgtaatgagagggctcatgagcagagctgcctatccctgggggttcactaacgcctacaggacatcctggcccaagtctgcctgcacaactaaaggcacacttctggtctttaggtccttcgctgtatgagcaagcaaaacctggagaatttcacttgcagaaaatccaccagttgctgcaatagttttatcatagtactacatttgaaaaaaaaatatttaaatagtaaaggagggagccatccaaatgaacaggaactgtggaaaggcagcaataactttatcagaagaatctattaccatctcagagtacaagcacatgcgcagacttttgtaatcaaagatgaaaattcttcaatttgtgtactgctaattttgttaagaaatataagccagccaatatgcttactttgaggccaaaggagcaaggtagtatgaggatgttaagacaccaagtactaaggatattaaggtaaactggtatgcagctgctagagggttcagttttgaaataaagcttagtcttatatccagacaggaagaggcagcacatgctaactttagcacgaaggacaagggtcttctcaaagagacagcctgctctttctcttcttgctctgagataaagtgccaaatagcagctttcaagttctagtgagagaaataaaaataaagctgggctactgcacatcaccaaacaaataggtattttcatatcgcatattacaaagtagaggttgagtatcccttatcagaaatgtttcggaccagaagtgttttggatttcagatgtttttgaaatttggaatatttgaaaaatacaaactggttgaacatcccaaatatgaaatccaaaatgctcaaatgagcatttcctttgagcatcatgtcggtattcaaaaagttttggattttggagcacttgattccaggagctcagcctgtatttagaaattaagcataacttctaaatagagctagctaatacttgctggttgcacttaagtatcatagtaattatcagcataaagtaaaaataagtatttactgcctaaaatgttgaaccaatgttttctgggaccatttctctaaatacacaaatggggagacatactagaaaaccttacaattaaatatgctggtagtgttagggttttagagcaaaacagaaatccaacccccaagaaagtcagggaaaagaagacaaaaatcagaagatgaacagctgcatatttctccacctaacactaggaggaaaaagtagaatatttgaaatacgatatggaatacaaatctgtgccatttagaacataatggtaggacgtagtaaacaagctacatcagcacaggacatggtttattgtcaaccatttaaacatataaacaaaactaagagtaagaaaataaaagacagatgctgtagcaaaagggcatttctctccaacatgattggccattattctccaaaatgtatggttaacagaaaattgaagaaaagtttgtatagagttattttaaatgattgatattttctggtttttttttttttttttttttttttttttgagacagggtcttgctctgtaatccaggctagagtgcaatggcatgatcacagctcattgcagccccaaacccccaggctcaaagtgatcctcctgcttcagcctcccgagtagctgggattaccaagcatgagccaccataccgagcaaatttaaaaaatttttttgtagagacagggtctctctatgttgctcaggctggttttgaactcctggactcaagcaatcctccctgcttcagcctcccaaagtgctgggattacaggcctccatgagcaaccacgcccagctcaagaatgattcacattttaattttcttttgaacaggtttaccactttgtatttgtgttttaggttttaagactaaatctgtgcaataatattccctagggattaaaagtaggggaaatacaaccctctccaaaagcagaaacaaaacttggggtggaaagaggaggtaaaaattacattcgcttttccaaatgagtctgaatcgtaaaaccataaagaatggttttactcattctttgtcagccatttgaaatcaataaactatgattcctacattttgtttgtattacacaaaaagtaaacaacaatgaaagctgtttttaaaagaataaaaaccaccaaccacaaatagaagagaaccccagacggttctcttggagggatgtttatcaccagtgccaaaagcctcccccctctgaaatgtttctctcagttgacaactttcaaatgatttaaagaacatgaagaacaagtagaacatgaagcttggatctgaatagtaaagaataatattggagtggtatttacaaaggagaggcagatatatgtgcctagcaccagatttttcaagtaagcaagttcagccccaaactaactgaagttttacatttttaaactctctccattatttcccagagttggaagctgtgaaatgtttcagcatggtgctattcactaatggtgtgaactcaaaaggtgggttttctgcagctgaactgattctaagtctcaggactccaagatacctccagtccaagtgtcgtggactctactggctttatacacctaatttgggactatccattttttccttctttaaagctggctagggaattccttcactaatgataatgtgtgcaaacacacacacatattgaaaatctataactaattctagcagccaaaagatgtttttccttaccagaaattacccaaagaaagttacattagaaataatatgactaaaaatatatttttaaagctatttaatactcatgatgtctaaactttcaatttattgtctgatttctggatatttctgtattttagattctacagacttcagattctgaagcttgttgaaaaagctaagttcctcaatatggatgaaaatctatctggctgtacttttagaggggaatttttctacttttgaaaaaaattctgaatatttatatatagtattaacagaataccccagtaagtcatatttcagataaatattctatagtataatttgcatcatacccaatattttagatattaaaataagggtaaaatttggaatataatcacttgtctgcatatttcccaatgtaagttttcatgtagaatattaaaatttaaattgatatttggatttataagctgttttccctgtatactatacgtatctattagcaatagagacaattttggagtcatggtatagtgaacctctctggctctccttgcacaaggctccatgagtcagtctgggcagtgcacgctacccttgcataactcactccccacactcaggcttaggggtactaacatgcaatcctaggacaacacttgacactagcactgacattttaaaattcattctcccaagtaataaaaaatatatatatagatagatatacacagagagatctgcagctgtactaattacttcaaatagcagcagacaaggaaaatacacgcttgcttgcttaagtttaaattcattttaagtttgctatattaaatttaaaaattaaaaaaatatcaacttactataaacaatttaaaatatgtataatacaacttcatggtcaaaacatttgaatagtctatgaaaacaggaaatacgttcatctgacatttctgtttagattccattcatgatttttcaatctgtctcttccaaaagaaaccataaagcagttgtcatattttatggcaactaattttgtttagggatttcctcatcacaaaaatactttatttcctattacaggggagttaaagaagaagaaaaaagaaatgagaaacaaagtggctttctccccacttgtcactattctcttcttcaaacattctgtacataagctgtctgagtcttttgaaccatttacaaattgtattttcaaaaattgaagaaaaaatatttagagtctaaaagtgttattttatacactgactatacaatatacattgaatgtttacacatacaaatacatcttaaagataaggttctccaaaggtttttcgacattccatcacccctgtacttggtggtctatcacagttgtgtgtactcttgacttgactaggtgtgagacgatcgtatgccatcttgtactctttatcaaaagcatctatatcaatgttttctcttcccagtgccacaagtgagagaaatagtatttctctgtataaactcctctgtcttttaaaatgtggacacttattcagtgtctctaaaatctgactcattggtccatagacatcattcattttaatgctttttaccatacttttcaacagttcctggttaaatgagttatcacttttttgcaataaatggaccattggatatttttgggtgtgtgcattccagagaatgtacaagggctgtcccggatcctgatgtaacttcatattgtcccataacatttgtattaaaacatatttgctatcttcagacatacagtggcggggaatctttgaatacttgttacagtgctcagaagaaagaatcaatccaggtaagttactgggcaagtcaagacgtctgaaataccataccaggttccaaaaaacaattggatgatggtccacaaagtctgctactgttattgcatgatcaccttcattttccaataagctttcaagttctttccataccactaaaggactaagatacggaacagtgacaggatcgggacttggaaggtgccattctaaacctaaagaatctgtagctccttgtaaagtagctggcaggctgcctgtagaaatgagcttctgtcttccagtatcttccttatccaaggggccagaagtactaatactcctggccattggaaatattggacatttagacatagctgtttttgatctattagcagggatctgaatacttcgggtgcaaaaattttcctgcagtttagatttgctatttagatcaaaattcccttgaacagagagagcagatgtgtcaagaccagaggctgatgttgaaatgcaagactgcctcgtctgacttgaaatggaggatggaaagtgcatattttctgttgatgggcttgactttagaaagtatcttccaggtcgtcttaaatctcttatttctatattcagaaagggtaagaagatattgccacagaatgggcatgtagtattgagatttgaatcatctgctgtccagccagccatgatttcctcatcatggacaagacaatcacaagttctacaccgagagcaacttgagatgagaacctccattgcatagttctggaagatatttgtattactcgcgttgaaggaagatgtcacttctgatttcccaggtaaggcaaacttcgacagagatccttccaaggatgcagaactttccaggcttattcggctgagatcaattctcttagtccctgaagtagcactggtctcttgagaggagataggtccttccaactcatggcagacatcttcatctgttaaagaggtagattcagaatcctgggctcccactgaagaaagactggtacgatcagaactttgatccttagatgatgtggtgtacatggtgaatcttgaataccatttgcttgctttctctgcaactccttttccagcagtgaacatactgtttcttagaacatctagtttaggtactagtagtgtatctaagttaaatgaaggtgatgagtgggttaatgtatcctgagattcttccctaaatgggcaagtaggtgagaaggctggagaagaccaaagtctatcccttggtttctcctcactttttgtgtaacttttagatttggtaagtctcactggcttaggagaattaggaggcagactagatcttctgcatgccttgaccaatggtggacttttcttatttaatttatcatcacatgcccgttgtaaatcaatgcttggtgtacgacttgtcaaaggactgctcatgttattcatatacatcacaatttcttcagctaaatcacgcctagcagatggtgttgaaatgcttttgctatcatcttcatcctcctcctcttcttctttttgctgctgttcagtctcagcaaccaaaagagagaggggatcaaatcctgttgcgacatcagttttttcaaaaggttttactgaaaagctgctgttcatacgttgaatcctcttgggattttgtgtagcaacacatcctgcttttgatacatctgtttcactgtctaagtcttctaagtcaaaaataacaggagaatccactttatctgccaaatagttagaaccatcaaaaggtgtatcatcatcactagattccttttctagactgtctctttttgatcttaaaggtggcttcccaatatcaagagtatttggtctcgtgctttttgagataacatttgaaagaatttttgcatcagctcccaatttttcaactatatctccaggggttgcttcctggttaattctattgagcataaatcccatcagtacccctccactaagattacggtttctatttccccagaccacttgctgctgcaaattagtttcattgtcacttttatgtcttttcctgaagcatctactttgaatgtttcgtgtttcatttgtatcttcaagagatgatattaagagcagctcaggtgtgctttccatgctttctcctgatattttaccagcactgttgttacttgtaccagtgaggcgaacgatactggaagaattttgataactgagcttaggaaggcaatcagcacttccttttgtactctcactctctgacaaggaactacaatcactcccttttttatctttttcttcttgaatgtcttcagtagatgtatcccctcttctaacttcatctttagataatgaattatatccaagatcagactggccacctgtactagatctatcatcagtagcatatactttgattaaacccgtattaaaaggtgcctgctccacagtgtgtgtcccatgaccactatccatgctgccatgactaacagcatccaggtcactgccatctgagagagttgtttgtgataagtgtgcatgcttctttaaagctcttttgaactgtgttactcctaaaacaacatttcttacttttgtccaaagaaaatagccactacgacttcttgaaggccaggtactttccaaaacagccttattataataaccataagtaatggcattggggtcaataccagctttctgcatttcaaaaagcactcgaactgcaagcactggctgatcatattgtccacagagttgcataagaatgcggtagcatacctcatcaggtggatccatcttctttgactgcatttttttaagcacatcatatgctgttttcagagccctgacttttgaatgacagactttcacataagctgggagacaaataaaccacagtccataacagtggcgcagtagacacctagaccacatctgagggatggaagagtacctctttgcaattttatgggctgatttaatttcctgttttgttcttctgaacatgggcaaagggctattaggactacttgattttgaaggcaatttgttcttctttgcttgtagaaatccttcaggtctttcaaataaattgttcctaagaactggaaatccattatagcacctaaaaattagggatctgtaaagtttggatttttgaaaataccacagtccttagaaagctacgtcacagatgatggattgcttctctctttcaatctcaaacattctgcctcttgaatacctgtactgtaaagggggttcttcaccattgggtaggtgggggatctcaggtggtgttacaaaaacagtgtgttcacttttgaaagattcatccagttctataagtcgtacttcaccgctcttgtccatatccactttatctacacaatcatcaaaaaatgccaggcttgcatctttgtcactaacaaaagaacattcttcaatgaagcgaataaacatttgtgttttggtcatcatgttatagaatttttgatgtgaccggtcccggcttcttaagaaagcttgtagggcaaagagagaggctgcatctgtggctgtctcagatggggcttgtgttattggccttaagtatgatctgtaaccttttaaaatagaggccatgaaaaacaaaaatgcctcttggatttccaaatctatcatgtgcaacctctttccagaattaaaatcatagtcatttattgctaaatccatgagtccatcatctctcggtctctgctgcaattttgccaattgctgatgcaaattattcagtgtgttcatcagatttttacatggcttctttggaagtatcttccaggctacatttttcttgtcaccaatttgagaaatagtgttggtatctacatcaacacaactgacatctggtggaggatcatagagatcaaagtatcttgaatcaatccctactatgaatggacatggtgcactcaagacatctgctaaagccagtgggcagagaggaacatacgggcatggccagtggaaagggaaaatcatagacactaatgcttctgtcacactagtaagcacggatggccgtagggaatggataagaattttatgttctgttactgcaaacaccagtagtgtcacagcattttcagggcctaaattctgcagtagtgttgaaaacttgccaccacttagtggaagaggtgaagacacaggctgactgagaatcagattatcatgtggtgataactgaactaaaatccgtggtctctgaggagatggaaaaggaactttatgcataaaatgagaaatatgcttctcaattggaaggacatgaggcccagagatggaataacgatacagaaaagtcagaaacttcctgaatgcatcaaaaaaaggccagtgagaaagaagacagatgcatttgttagtatgaattgttttggaactatcagacttcccatctgctgatgttaaacccaaaagaagtctctgcttttctgtgagattctcctcagagtatggttcataaaactgaatagcagcaccataaaccttttcagctgaggctccagttaaaacaaaagtagaaaatacaggcagagggtatttgctatttgatggccaacattcaatggttgcacccattggtaaacaaaatagaggaacagattccggtagtgagaatgactcataatcttcttgaggatatctacaaattaggccagctttgtaagatacagtgttcgtctttgccaccgattttttataacacaagtatactgctgatccccacatactgttattgagattcttgtcgactttgcagaacgtgtgtggtgggctttctcctttactgggtataataatacatatgtcagtgacagccaacgtattctgagtcatgttttcagaggctcttcggtaagtgatataaattctttgtgatgaggtactcccactaatatttgcggggcgcccatagggagtactctgaataatttcacaaccctgtttcaatctttctttccagtcatataaaacccccagatctgtaagtggaggcttatctcttcctcttctatagcaaaggtaaatctgtggccccacaagacttccattattaagatcagctgacaatccagttggggtaacatcaatacagatataatcctgtgggacttcctccccaagagatttgataataactgaaacatctgtaataggttcttttggtttagctactttatgacaagcatcattgaagtgaatttcttcttctagaggctttgaaacatcagttaatcctgctacaacaaagtagtcagcaacacgaggccccttgtcttcaatcatcttccattacagaaggttacatacattaccgaaagtttctctctgaaaaagatgacagatttcaatgtgtgaactccgcagcctcagagtttgagaaataacacccagctggctcccgtgcgagcagcggatcgagctcggagagcggcgccggaatcccgcacgcgcggtagcggaacacgaggggctgaat

SEQ ID NO: 15512 - RNA, 10755 nt, Homo sapiens
  source 1..10755: mol_type = other RNA
gctgggattacaggcatgagccactgtacccagccaaaatggttactatatattttgaacattatattgcactgtcatcaatagattcgaaaatagttttaccaaattacaggcttagtcttttatagctgtctatatcaatattatttaaagattgagtaccaaagggggcaggaattggaatgtattatctagagcacagaatagtaaataatcaggaaaagggccgggcgcggtggctcatgcctataatcccagcactttgggaggccaaggtgggcggatcacgaggtcagtagatcgagaccatcctggctaacacggtgaaaccccgtctctactaaaaaaataccaaaaattagccgggcgaggtggcaggcgcctatagtcccagctactcgggaggctgaggcaggagaatggcgtgaaccccggggggcggagcctgcagtgagccgagatcgtgccactgcactccagcctgggcaacagcgagactccgtctcaaaaaaaaagaaaaaataaataatcaggaagaattggttggccttatgtgccaatgaatactcttggttctgacccttttttggtgggagggtcctccagcaggtgcagcttgcaatgtgtacggggactggatgctatgaaagatgtaatgagagggctcatgagcagagctgcctatccctgggggttcactaacgcctacaggacatcctggcccaagtctgcctgcacaactaaaggcacacttctggtctttaggtccttcgctgtatgagcaagcaaaacctggagaatttcacttgcagaaaatccaccagttgctgcaatagttttatcatagtactacatttgaaaaaaaaatatttaaatagtaaaggagggagccatccaaatgaacaggaactgtggaaaggcagcaataactttatcagaagaatctattaccatctcagagtacaagcacatgcgcagacttttgtaatcaaagatgaaaattcttcaatttgtgtactgctaattttgttaagaaatataagccagccaatatgcttactttgaggccaaaggagcaaggtagtatgaggatgttaagacaccaagtactaaggatattaaggtaaactggtatgcagctgctagagggttcagttttgaaataaagcttagtcttatatccagacaggaagaggcagcacatgctaactttagcacgaaggacaagggtcttctcaaagagacagcctgctctttctcttcttgctctgagataaagtgccaaatagcagctttcaagttctagtgagagaaataaaaataaagctgggctactgcacatcaccaaacaaataggtattttcatatcgcatattacaaagtagaggttgagtatcccttatcagaaatgtttcggaccagaagtgttttggatttcagatgtttttgaaatttggaatatttgaaaaatacaaactggttgaacatcccaaatatgaaatccaaaatgctcaaatgagcatttcctttgagcatcatgtcggtattcaaaaagttttggattttggagcacttgattccaggagctcagcctgtatttagaaattaagcataacttctaaatagagctagctaatacttgctggttgcacttaagtatcatagtaattatcagcataaagtaaaaataagtatttactgcctaaaatgttgaaccaatgttttctgggaccatttctctaaatacacaaatggggagacatactagaaaaccttacaattaaatatgctggtagtgttagggttttagagcaaaacagaaatccaacccccaagaaagtcagggaaaagaagacaaaaatcagaagatgaacagctgcatatttctccacctaacactaggaggaaaaagtagaatatttgaaatacgatatggaatacaaatctgtgccatttagaacataatggtaggacgtagtaaacaagctacatcagcacaggacatggtttattgtcaaccatttaaacatataaacaaaactaagagtaagaaaataaaagacagatgctgtagcaaaagggcatttctctccaacatgattggccattattctccaaaatgtatggttaacagaaaattgaagaaaagtttgtatagagttattttaaatgattgatattttctggtttttttttttttttttttttttttttttgagacagggtcttgctctgtaatccaggctagagtgcaatggcatgatcacagctcattgcagccccaaacccccaggctcaaagtgatcctcctgcttcagcctcccgagtagctgggattaccaagcatgagccaccataccgagcaaatttaaaaaatttttttgtagagacagggtctctctatgttgctcaggctggttttgaactcctggactcaagcaatcctccctgcttcagcctcccaaagtgctgggattacaggcctccatgagcaaccacgcccagctcaagaatgattcacattttaattttcttttgaacaggtttaccactttgtatttgtgttttaggttttaagactaaatctgtgcaataatattccctagggattaaaagtaggggaaatacaaccctctccaaaagcagaaacaaaacttggggtggaaagaggaggtaaaaattacattcgcttttccaaatgagtctgaatcgtaaaaccataaagaatggttttactcattctttgtcagccatttgaaatcaataaactatgattcctacattttgtttgtattacacaaaaagtaaacaacaatgaaagctgtttttaaaagaataaaaaccaccaaccacaaatagaagagaaccccagacggttctcttggagggatgtttatcaccagtgccaaaagcctcccccctctgaaatgtttctctcagttgacaactttcaaatgatttaaagaacatgaagaacaagtagaacatgaagcttggatctgaatagtaaagaataatattggagtggtatttacaaaggagaggcagatatatgtgcctagcaccagatttttcaagtaagcaagttcagccccaaactaactgaagttttacatttttaaactctctccattatttcccagagttggaagctgtgaaatgtttcagcatggtgctattcactaatggtgtgaactcaaaaggtgggttttctgcagctgaactgattctaagtctcaggactccaagatacctccagtccaagtgtcgtggactctactggctttatacacctaatttgggactatccattttttccttctttaaagctggctagggaattccttcactaatgataatgtgtgcaaacacacacacatattgaaaatctataactaattctagcagccaaaagatgtttttccttaccagaaattacccaaagaaagttacattagaaataatatgactaaaaatatatttttaaagctatttaatactcatgatgtctaaactttcaatttattgtctgatttctggatatttctgtattttagattctacagacttcagattctgaagcttgttgaaaaagctaagttcctcaatatggatgaaaatctatctggctgtacttttagaggggaatttttctacttttgaaaaaaattctgaatatttatatatagtattaacagaataccccagtaagtcatatttcagataaatattctatagtataatttgcatcatacccaatattttagatattaaaataagggtaaaatttggaatataatcacttgtctgcatatttcccaatgtaagttttcatgtagaatattaaaatttaaattgatatttggatttataagctgttttccctgtatactatacgtatctattagcaatagagacaattttggagtcatggtatagtgaacctctctggctctccttgcacaaggctccatgagtcagtctgggcagtgcacgctacccttgcataactcactccccacactcaggcttaggggtactaacatgcaatcctaggacaacacttgacactagcactgacattttaaaattcattctcccaagtaataaaaaatatatatatagatagatatacacagagagatctgcagctgtactaattacttcaaatagcagcagacaaggaaaatacacgcttgcttgcttaagtttaaattcattttaagtttgctatattaaatttaaaaattaaaaaaatatcaacttactataaacaatttaaaatatgtataatacaacttcatggtcaaaacatttgaatagtctatgaaaacaggaaatacgttcatctgacatttctgtttagattccattcatgatttttcaatctgtctcttccaaaagaaaccataaagcagttgtcatattttatggcaactaattttgtttagggatttcctcatcacaaaaatactttatttcctattacaggggagttaaagaagaagaaaaaagaaatgagaaacaaagtggctttctccccacttgtcactattctcttcttcaaacattctgtacataagctgtctgagtcttttgaaccatttacaaattgtattttcaaaaattgaagaaaaaatatttagagtctaaaagtgttattttatacactgactatacaatatacattgaatgtttacacatacaaatacatcttaaagataaggttctccaaaggtttttcgacattccatcacccctgtacttggtggtctatcacagttgtgtgtactcttgacttgactaggtgtgagacgatcgtatgccatcttgtactctttatcaaaagcatctatatcaatgttttctcttcccagtgccacaagtgagagaaatagtatttctctgtataaactcctctgtcttttaaaatgtggacacttattcagtgtctctaaaatctgactcattggtccatagacatcattcattttaatgctttttaccatacttttcaacagttcctggttaaatgagttatcacttttttgcaataaatggaccattggatatttttgggtgtgtgcattccagagaatgtacaagggctgtcccggatcctgatgtaacttcatattgtcccataacatttgtattaaaacatatttgctatcttcagacatacagtggcggggaatctttgaatacttgttacagtgctcagaagaaagaatcaatccaggtaagttactgggcaagtcaagacgtctgaaataccataccaggttccaaaaaacaattggatgatggtccacaaagtctgctactgttattgcatgatcaccttcattttccaataagctttcaagttctttccataccactaaaggactaagatacggaacagtgacaggatcgggacttggaaggtgccattctaaacctaaagaatctgtagctccttgtaaagtagctggcaggctgcctgtagaaatgagcttctgtcttccagtatcttccttatccaaggggccagaagtactaatactcctggccattggaaatattggacatttagacatagctgtttttgatctattagcagggatctgaatacttcgggtgcaaaaattttcctgcagtttagatttgctatttagatcaaaattcccttgaacagagagagcagatgtgtcaagaccagaggctgatgttgaaatgcaagactgcctcgtctgacttgaaatggaggatggaaagtgcatattttctgttgatgggcttgactttagaaagtatcttccaggtcgtcttaaatctcttatttctatattcagaaagggtaagaagatattgccacagaatgggcatgtagtattgagatttgaatcatctgctgtccagccagccatgatttcctcatcatggacaagacaatcacaagttctacaccgagagcaacttgagatgagaacctccattgcatagttctggaagatatttgtattactcgcgttgaaggaagatgtcacttctgatttcccaggtaaggcaaacttcgacagagatccttccaaggatgcagaactttccaggcttattcggctgagatcaattctcttagtccctgaagtagcactggtctcttgagaggagataggtccttccaactcatggcagacatcttcatctgttaaagaggtagattcagaatcctgggctcccactgaagaaagactggtacgatcagaactttgatccttagatgatgtggtgtacatggtgaatcttgaataccatttgcttgctttctctgcaactccttttccagcagtgaacatactgtttcttagaacatctagtttaggtactagtagtgtatctaagttaaatgaaggtgatgagtgggttaatgtatcctgagattcttccctaaatgggcaagtaggtgagaaggctggagaagaccaaagtctatcccttggtttctcctcactttttgtgtaacttttagatttggtaagtctcactggcttaggagaattaggaggcagactagatcttctgcatgccttgaccaatggtggacttttcttatttaatttatcatcacatgcccgttgtaaatcaatgcttggtgtacgacttgtcaaaggactgctcatgttattcatatacatcacaatttcttcagctaaatcacgcctagcagatggtgttgaaatgcttttgctatcatcttcatcctcctcctcttcttctttttgctgctgttcagtctcagcaaccaaaagagagaggggatcaaatcctgttgcgacatcagttttttcaaaaggttttactgaaaagctgctgttcatacgttgaatcctcttgggattttgtgtagcaacacatcctgcttttgatacatctgtttcactgtctaagtcttctaagtcaaaaataacaggagaatccactttatctgccaaatagttagaaccatcaaaaggtgtatcatcatcactagattccttttctagactgtctctttttgatcttaaaggtggcttcccaatatcaagagtatttggtctcgtgctttttgagataacatttgaaagaatttttgcatcagctcccaatttttcaactatatctccaggggttgcttcctggttaattctattgagcataaatcccatcagtacccctccactaagattacggtttctatttccccagaccacttgctgctgcaaattagtttcattgtcacttttatgtcttttcctgaagcatctactttgaatgtttcgtgtttcatttgtatcttcaagagatgatattaagagcagctcaggtgtgctttccatgctttctcctgatattttaccagcactgttgttacttgtaccagtgaggcgaacgatactggaagaattttgataactgagcttaggaaggcaatcagcacttccttttgtactctcactctctgacaaggaactacaatcactcccttttttatctttttcttcttgaatgtcttcagtagatgtatcccctcttctaacttcatctttagataatgaattatatccaagatcagactggccacctgtactagatctatcatcagtagcatatactttgattaaacccgtattaaaaggtgcctgctccacagtgtgtgtcccatgaccactatccatgctgccatgactaacagcatccaggtcactgccatctgctgagagagttgtttgtgataagtgtgcatgcttctttaaagctcttttgaactgtgttactcctaaaacaacatttcttacttttgtccaaagaaaatagccactacgacttcttgaaggccaggtactttccaaaacagccttattataataaccataagtaatggcattggggtcaataccagctttctgcatttcaaaaagcactcgaactgcaagcactggctgatcatattgtccacagagttgcataagaatgcggtagcatacctcatcaggtggatccatcttctttgactgcatttttttaagcacatcatatgctgttttcagagccctgacttttgaatgacagactttcacataagctgggagacaaataaaccacagtccataacagtggcgcagtagacacctagaccacatctgagggatggaagagtacctctttgcaattttatgggctgatttaatttcctgttttgttcttctgaacatgggcaaagggctattaggactacttgattttgaaggcaatttgttcttctttgcttgtagaaatccttcaggtctttcaaataaattgttcctaagaactggaaatccattatagcacctaaaaattagggatctgtaaagtttggatttttgaaaataccacagtccttagaaagctacgtcacagatgatggattgcttctctctttcaatctcaaacattctgcctcttgaatacctgtactgtaaagggggttcttcaccattgggtaggtgggggatctcaggtggtgttacaaaaacagtgtgttcacttttgaaagattcatccagttctataagtcgtacttcaccgctcttgtccatatccactttatctacacaatcatcaaaaaatgccaggcttgcatctttgtcactaacaaaagaacattcttcaatgaagcgaataaacatttgtgttttggtcatcatgttatagaatttttgatgtgaccggtcccggcttcttaagaaagcttgtagggcaaagagagaggctgcatctgtggctgtctcagatggggcttgtgttattggccttaagtatgatctgtaaccttttaaaatagaggccatgaaaaacaaaaatgcctcttggatttccaaatctatcatgtgcaacctctttccagaattaaaatcatagtcatttattgctaaatccatgagtccatcatctctcggtctctgctgcaattttgccaattgctgatgcaaattattcagtgtgttcatcagatttttacatggcttctttggaagtatcttccaggctacatttttcttgtcaccaatttgagaaatagtgttggtatctacatcaacacaactgacatctggtggaggatcatagagatcaaagtatcttgaatcaatccctactatgaatggacatggtgcactcaagacatctgctaaagccagtgggcagagaggaacatacgggcatggccagtggaaagggaaaatcatagacactaatgcttctgtcacactagtaagcacggatggccgtagggaatggataagaattttatgttctgttactgcaaacaccagtagtgtcacagcattttcagggcctaaattctgcagtagtgttgaaaacttgccaccacttagtggaagaggtgaagacacaggctgactgagaatcagattatcatgtggtgataactgaactaaaatccgtggtctctgaggagatggaaaaggaactttatgcataaaatgagaaatatgcttctcaattggaaggacatgaggcccagagatggaataacgatacagaaaagtcagaaacttcctgaatgcatcaaaaaaaggccagtgagaaagaagacagatgcatttgttagtatgaattgttttggaactatcagacttcccatctgctgatgttaaacccaaaagaagtctctgcttttctgtgagattctcctcagagtatggttcataaaactgaatagcagcaccataaaccttttcagctgaggctccagttaaaacaaaagtagaaaatacaggcagagggtatttgctatttgatggccaacattcaatggttgcacccattggtaaacaaaatagaggaacagattccggtagtgagaatgactcataatcttcttgaggatatctacaaattaggccagctttgtaagatacagtgttcgtctttgccaccgattttttataacacaagtatactgctgatccccacatactgttattgagattcttgtcgactttgcagaacgtgtgtggtgggctttctcctttactgggtataataatacatatgtcagtgacagccaacgtattctgagtcatgttttcagaggctcttcggtaagtgatataaattctttgtgatgaggtactcccactaatatttgcggggcgcccatagggagtactctgaataatttcacaaccctgtttcaatctttctttccagtcatataaaacccccagatctgtaagtggaggcttatctcttcctcttctatagcaaaggtaaatctgtggccccacaagacttccattattaagatcagctgacaatccagttggggtaacatcaatacagatataatcctgtgggacttcctccccaagagatttgataataactgaaacatctgtaataggttcttttggtttagctactttatgacaagcatcattgaagtgaatttcttcttctagaggctttgaaacatcagttaatcctgctacaacaaagtagtcagcaacacgaggccccttgtcttcaatcatcttccattacagaaggttacatacattaccgaaagtttctctctgaaaaagatgacagatttcaatgtgtgaactccgcagcctcagagtttgagaaataacacccagctggctcccgtgcgagcagcggatcgagctcggagagcggcgccggaatcccgcacgcgcggtagcggaacacgaggggctgaat

SEQ ID NO: 15513 - RNA, 10559 nt, Homo sapiens
  source 1..10559: mol_type = other RNA
gctgggattacaggcatgagccactgtacccagccaaaatggttactatatattttgaacattatattgcactgtcatcaatagattcgaaaatagttttaccaaattacaggcttagtcttttatagctgtctatatcaatattatttaaagattgagtaccaaagggggcaggaattggaatgtattatctagagcacagaatagtaaataatcaggaaaagggccgggcgcggtggctcatgcctataatcccagcactttgggaggccaaggtgggcggatcacgaggtcagtagatcgagaccatcctggctaacacggtgaaaccccgtctctactaaaaaaataccaaaaattagccgggcgaggtggcaggcgcctatagtcccagctactcgggaggctgaggcaggagaatggcgtgaaccccggggggcggagcctgcagtgagccgagatcgtgccactgcactccagcctgggcaacagcgagactccgtctcaaaaaaaaagaaaaaataaataatcaggaagaattggttggccttatgtgccaatgaatactcttggttctgacccttttttggtgggagggtcctccagcaggtgcagcttgcaatgtgtacggggactggatgctatgaaagatgtaatgagagggctcatgagcagagctgcctatccctgggggttcactaacgcctacaggacatcctggcccaagtctgcctgcacaactaaaggcacacttctggtctttaggtccttcgctgtatgagcaagcaaaacctggagaatttcacttgcagaaaatccaccagttgctgcaatagttttatcatagtactacatttgaaaaaaaaatatttaaatagtaaaggagggagccatccaaatgaacaggaactgtggaaaggcagcaataactttatcagaagaatctattaccatctcagagtacaagcacatgcgcagacttttgtaatcaaagatgaaaattcttcaatttgtgtactgctaattttgttaagaaatataagccagccaatatgcttactttgaggccaaaggagcaaggtagtatgaggatgttaagacaccaagtactaaggatattaaggtaaactggtatgcagctgctagagggttcagttttgaaataaagcttagtcttatatccagacaggaagaggcagcacatgctaactttagcacgaaggacaagggtcttctcaaagagacagcctgctctttctcttcttgctctgagataaagtgccaaatagcagctttcaagttctagtgagagaaataaaaataaagctgggctactgcacatcaccaaacaaataggtattttcatatcgcatattacaaagtagaggttgagtatcccttatcagaaatgtttcggaccagaagtgttttggatttcagatgtttttgaaatttggaatatttgaaaaatacaaactggttgaacatcccaaatatgaaatccaaaatgctcaaatgagcatttcctttgagcatcatgtcggtattcaaaaagttttggattttggagcacttgattccaggagctcagcctgtatttagaaattaagcataacttctaaatagagctagctaatacttgctggttgcacttaagtatcatagtaattatcagcataaagtaaaaataagtatttactgcctaaaatgttgaaccaatgttttctgggaccatttctctaaatacacaaatggggagacatactagaaaaccttacaattaaatatgctggtagtgttagggttttagagcaaaacagaaatccaacccccaagaaagtcagggaaaagaagacaaaaatcagaagatgaacagctgcatatttctccacctaacactaggaggaaaaagtagaatatttgaaatacgatatggaatacaaatctgtgccatttagaacataatggtaggacgtagtaaacaagctacatcagcacaggacatggtttattgtcaaccatttaaacatataaacaaaactaagagtaagaaaataaaagacagatgctgtagcaaaagggcatttctctccaacatgattggccattattctccaaaatgtatggttaacagaaaattgaagaaaagtttgtatagagttattttaaatgattgatattttctggtttttttttttttttttttttttttttttgagacagggtcttgctctgtaatccaggctagagtgcaatggcatgatcacagctcattgcagccccaaacccccaggctcaaagtgatcctcctgcttcagcctcccgagtagctgggattaccaagcatgagccaccataccgagcaaatttaaaaaatttttttgtagagacagggtctctctatgttgctcaggctggttttgaactcctggactcaagcaatcctccctgcttcagcctcccaaagtgctgggattacaggcctccatgagcaaccacgcccagctcaagaatgattcacattttaattttcttttgaacaggtttaccactttgtatttgtgttttaggttttaagactaaatctgtgcaataatattccctagggattaaaagtaggggaaatacaaccctctccaaaagcagaaacaaaacttggggtggaaagaggaggtaaaaattacattcgcttttccaaatgagtctgaatcgtaaaaccataaagaatggttttactcattctttgtcagccatttgaaatcaataaactatgattcctacattttgtttgtattacacaaaaagtaaacaacaatgaaagctgtttttaaaagaataaaaaccaccaaccacaaatagaagagaaccccagacggttctcttggagggatgtttatcaccagtgccaaaagcctcccccctctgaaatgtttctctcagttgacaactttcaaatgatttaaagaacatgaagaacaagtagaacatgaagcttggatctgaatagtaaagaataatattggagtggtatttacaaaggagaggcagatatatgtgcctagcaccagatttttcaagtaagcaagttcagccccaaactaactgaagttttacatttttaaactctctccattatttcccagagttggaagctgtgaaatgtttcagcatggtgctattcactaatggtgtgaactcaaaaggtgggttttctgcagctgaactgattctaagtctcaggactccaagatacctccagtccaagtgtcgtggactctactggctttatacacctaatttgggactatccattttttccttctttaaagctggctagggaattccttcactaatgataatgtgtgcaaacacacacacatattgaaaatctataactaattctagcagccaaaagatgtttttccttaccagaaattacccaaagaaagttacattagaaataatatgactaaaaatatatttttaaagctatttaatactcatgatgtctaaactttcaatttattgtctgatttctggatatttctgtattttagattctacagacttcagattctgaagcttgttgaaaaagctaagttcctcaatatggatgaaaatctatctggctgtacttttagaggggaatttttctacttttgaaaaaaattctgaatatttatatatagtattaacagaataccccagtaagtcatatttcagataaatattctatagtataatttgcatcatacccaatattttagatattaaaataagggtaaaatttggaatataatcacttgtctgcatatttcccaatgtaagttttcatgtagaatattaaaatttaaattgatatttggatttataagctgttttccctgtatactatacgtatctattagcaatagagacaattttggagtcatggtatagtgaacctctctggctctccttgcacaaggctccatgagtcagtctgggcagtgcacgctacccttgcataactcactccccacactcaggcttaggggtactaacatgcaatcctaggacaacacttgacactagcactgacattttaaaattcattctcccaagtaataaaaaatatatatatagatagatatacacagagagatctgcagctgtactaattacttcaaatagcagcagacaaggaaaatacacgcttgcttgcttaagtttaaattcattttaagtttgctatattaaatttaaaaattaaaaaaatatcaacttactataaacaatttaaaatatgtataatacaacttcatggtcaaaacatttgaatagtctatgaaaacaggaaatacgttcatctgacatttctgtttagattccattcatgatttttcaatctgtctcttccaaaagaaaccataaagcagttgtcatattttatggcaactaattttgtttagggatttcctcatcacaaaaatactttatttcctattacaggggagttaaagaagaagaaaaaagaaatgagaaacaaagtggctttctccccacttgtcactattctcttcttcaaacattctgtacataagctgtctgagtcttttgaaccatttacaaattgtattttcaaaaattgaagaaaaaatatttagagtctaaaagtgttattttatacactgactatacaatatacattgaatgtttacacatacaaatacatcttaaagataaggttctccaaaggtttttcgacattccatcacccctgtacttggtggtctatcacagttgtgtgtactcttgacttgactaggtgtgagacgatcgtatgccatcttgtactctttatcaaaagcatctatatcaatgttttctcttcccagtgccacaagtgagagaaatagtatttctctgtataaactcctctgtcttttaaaatgtggacacttattcagtgtctctaaaatctgactcattggtccatagacatcattcattttaatgctttttaccatacttttcaacagttcctggttaaatgagttatcacttttttgcaataaatggaccattggatatttttgggtgtgtgcattccagagaatgtacaagggctgtcccggatcctgatgtaacttcatattgtcccataacatttgtattaaaacatatttgctatcttcagacatacagtggcggggaatctttgaatacttgttacagtgctcagaagaaagaatcaatccaggtaagttactgggcaagtcaagacgtctgaaataccataccaggttccaaaaaacaattggatgatggtccacaaagtctgctactgttattgcatgatcaccttcattttccaataagctttcaagttctttccataccactaaaggactaagatacggaacagtgacaggatcgggacttggaaggtgccattctaaacctaaagaatctgtagctccttgtaaagtagctggcaggctgcctgtagaaatgagcttctgtcttccagtatcttccttatccaaggggccagaagtactaatactcctggccattggaaatattggacatttagacatagctgtttttgatctattagcagggatctgaatacttcgggtgcaaaaattttcctgcagtttagatttgctatttagatcaaaattcccttgaacagagagagcagatgtgtcaagaccagaggctgatgttgaaatgcaagactgcctcgtctgacttgaaatggaggatggaaagtgcatattttctgttgatgggcttgactttagaaagtatcttccaggtcgtcttaaatctcttatttctatattcagaaagggtaagaagatattgccacagaatgggcatgtagtattgagatttgaatcatctgctgtccagccagccatgatttcctcatcatggacaagacaatcacaagttctacaccgagagcaacttgagatgagaacctccattgcatagttctggaagatatttgtattactcgcgttgaaggaagatgtcacttctgatttcccaggtaaggcaaacttcgacagagatccttccaaggatgcagaactttccaggcttattcggctgagatcaattctcttagtccctgaagtagcactggtctcttgagaggagataggtccttccaactcatggcagacatcttcatctgttaaagaggtagattcagaatcctgggctcccactgaagaaagactggtacgatcagaactttgatccttagatgatgtggtgtacatggtgaatcttgaataccatttgcttgctttctctgcaactccttttccagcagtgaacatactgtttcttagaacatctagtttaggtactagtagtgtatctaagttaaatgaaggtgatgagtgggttaatgtatcctgagattcttccctaaatgggcaagtaggtgagaaggctggagaagaccaaagtctatcccttggtttctcctcactttttgtgtaacttttagatttggtaagtctcactggcttaggagaattaggaggcagactagatcttctgcatgccttgaccaatggtggacttttcttatttaatttatcatcacatgcccgttgtaaatcaatgcttggtgtacgacttgtcaaaggactgctcatgttattcatatacatcacaatttcttcagctaaatcacgcctagcagatggtgttgaaatgcttttgctatcatcttcatcctcctcctcttcttctttttgctgctgttcagtctcagcaaccaaaagagagaggggatcaaatcctgttgcgacatcagttttttcaaaaggttttactgaaaagctgctgttcatacgttgaatcctcttgggattttgtgtagcaacacatcctgcttttgatacatctgtttcactgtctaagtcttctaagtcaaaaataacaggagaatccactttatctgccaaatagttagaaccatcaaaaggtgtatcatcatcactagattccttttctagactgtctctttttgatcttaaaggtggcttcccaatatcaagagtatttggtctcgtgctttttgagataacatttgaaagaatttttgcatcagctcccaatttttcaactatatctccaggggttgcttcctggttaattctattgagcataaatcccatcagtacccctccactaagattacggtttctatttccccagaccacttgctgctgcaaattagtttcattgtcacttttatgtcttttcctgaagcatctactttgaatgtttcgtgtttcatttgtatcttcaagagatgatattaagagcagctcaggtgtgctttccatgctttctcctgatattttaccagcactgttgttacttgtaccagtgaggcgaacgatactggaagaattttgataactgagcttaggaaggcaatcagcacttccttttgtactctcactctctgacaaggaactacaatcactcccttttttatctttttcttcttgaatgtcttcagtagatgtatcccctcttctaacttcatctttagataatgaattatatccaagatcagactggccacctgtactagatctatcatcagtagcatatactttgattaaacccgtattaaaaggtgcctgctccacagtgtgtgtcccatgaccactatccatgctgccatgactaacagcatccaggtcactgccatctgctgagagagttgtttgtgataagtgtgcatgcttctttaaagctcttttgaactgtgttactcctaaaacaacatttcttacttttgtccaaagaaaatagccactacgacttcttgaaggccaggtactttccaaaacagccttattataataaccataagtaatggcattggggtcaataccagctttctgcatttcaaaaagcactcgaactgcaagcactggctgatcatattgtccacagagttgcataagaatgcggtagcatacctcatcaggtggatccatcttctttgactgcatttttttaagcacatcatatgctgttttcagagccctgacttttgaatgacagactttcacataagctgggagacaaataaaccacagtccataacagtggcgcagtagacacctagaccacatctgagggatggaagagtacctctttgcaattttatgggctgatttaatttcctgttttgttcttctgaacatgggcaaagggctattaggactacttgattttgaaggcaatttgttcttctttgcttgtagaaatccttcaggtctttcaaataaattgttcctaagaactggaaatccattatagctgtactgtaaagggggttcttcaccattgggtaggtgggggatctcaggtggtgttacaaaaacagtgtgttcacttttgaaagattcatccagttctataagtcgtacttcaccgctcttgtccatatccactttatctacacaatcatcaaaaaatgccaggcttgcatctttgtcactaacaaaagaacattcttcaatgaagcgaataaacatttgtgttttggtcatcatgttatagaatttttgatgtgaccggtcccggcttcttaagaaagcttgtagggcaaagagagaggctgcatctgtggctgtctcagatggggcttgtgttattggccttaagtatgatctgtaaccttttaaaatagaggccatgaaaaacaaaaatgcctcttggatttccaaatctatcatgtgcaacctctttccagaattaaaatcatagtcatttattgctaaatccatgagtccatcatctctcggtctctgctgcaattttgccaattgctgatgcaaattattcagtgtgttcatcagatttttacatggcttctttggaagtatcttccaggctacatttttcttgtcaccaatttgagaaatagtgttggtatctacatcaacacaactgacatctggtggaggatcatagagatcaaagtatcttgaatcaatccctactatgaatggacatggtgcactcaagacatctgctaaagccagtgggcagagaggaacatacgggcatggccagtggaaagggaaaatcatagacactaatgcttctgtcacactagtaagcacggatggccgtagggaatggataagaattttatgttctgttactgcaaacaccagtagtgtcacagcattttcagggcctaaattctgcagtagtgttgaaaacttgccaccacttagtggaagaggtgaagacacaggctgactgagaatcagattatcatgtggtgataactgaactaaaatccgtggtctctgaggagatggaaaaggaactttatgcataaaatgagaaatatgcttctcaattggaaggacatgaggcccagagatggaataacgatacagaaaagtcagaaacttcctgaatgcatcaaaaaaaggccagtgagaaagaagacagatgcatttgttagtatgaattgttttggaactatcagacttcccatctgctgatgttaaacccaaaagaagtctctgcttttctgtgagattctcctcagagtatggttcataaaactgaatagcagcaccataaaccttttcagctgaggctccagttaaaacaaaagtagaaaatacaggcagagggtatttgctatttgatggccaacattcaatggttgcacccattggtaaacaaaatagaggaacagattccggtagtgagaatgactcataatcttcttgaggatatctacaaattaggccagctttgtaagatacagtgttcgtctttgccaccgattttttataacacaagtatactgctgatccccacatactgttattgagattcttgtcgactttgcagaacgtgtgtggtgggctttctcctttactgggtataataatacatatgtcagtgacagccaacgtattctgagtcatgttttcagaggctcttcggtaagtgatataaattctttgtgatgaggtactcccactaatatttgcggggcgcccatagggagtactctgaataatttcacaaccctgtttcaatctttctttccagtcatataaaacccccagatctgtaagtggaggcttatctcttcctcttctatagcaaaggtaaatctgtggccccacaagacttccattattaagatcagctgacaatccagttggggtaacatcaatacagatataatcctgtgggacttcctccccaagagatttgataataactgaaacatctgtaataggttcttttggtttagctactttatgacaagcatcattgaagtgaatttcttcttctagaggctttgaaacatcagttaatcctgctacaacaaagtagtcagcaacacgaggccccttgtcttcaatcatcttccattacagaaggttacatacattaccgaaagtttctctctgaaaaagatgacagatttcaatgtgtgaactccgcagcctcagagtttgagaaataactctccgggccgtgacagc

SEQ ID NO: 15514 - RNA, 10602 nt, Homo sapiens
  source 1..10602: mol_type = other RNA
gctgggattacaggcatgagccactgtacccagccaaaatggttactatatattttgaacattatattgcactgtcatcaatagattcgaaaatagttttaccaaattacaggcttagtcttttatagctgtctatatcaatattatttaaagattgagtaccaaagggggcaggaattggaatgtattatctagagcacagaatagtaaataatcaggaaaagggccgggcgcggtggctcatgcctataatcccagcactttgggaggccaaggtgggcggatcacgaggtcagtagatcgagaccatcctggctaacacggtgaaaccccgtctctactaaaaaaataccaaaaattagccgggcgaggtggcaggcgcctatagtcccagctactcgggaggctgaggcaggagaatggcgtgaaccccggggggcggagcctgcagtgagccgagatcgtgccactgcactccagcctgggcaacagcgagactccgtctcaaaaaaaaagaaaaaataaataatcaggaagaattggttggccttatgtgccaatgaatactcttggttctgacccttttttggtgggagggtcctccagcaggtgcagcttgcaatgtgtacggggactggatgctatgaaagatgtaatgagagggctcatgagcagagctgcctatccctgggggttcactaacgcctacaggacatcctggcccaagtctgcctgcacaactaaaggcacacttctggtctttaggtccttcgctgtatgagcaagcaaaacctggagaatttcacttgcagaaaatccaccagttgctgcaatagttttatcatagtactacatttgaaaaaaaaatatttaaatagtaaaggagggagccatccaaatgaacaggaactgtggaaaggcagcaataactttatcagaagaatctattaccatctcagagtacaagcacatgcgcagacttttgtaatcaaagatgaaaattcttcaatttgtgtactgctaattttgttaagaaatataagccagccaatatgcttactttgaggccaaaggagcaaggtagtatgaggatgttaagacaccaagtactaaggatattaaggtaaactggtatgcagctgctagagggttcagttttgaaataaagcttagtcttatatccagacaggaagaggcagcacatgctaactttagcacgaaggacaagggtcttctcaaagagacagcctgctctttctcttcttgctctgagataaagtgccaaatagcagctttcaagttctagtgagagaaataaaaataaagctgggctactgcacatcaccaaacaaataggtattttcatatcgcatattacaaagtagaggttgagtatcccttatcagaaatgtttcggaccagaagtgttttggatttcagatgtttttgaaatttggaatatttgaaaaatacaaactggttgaacatcccaaatatgaaatccaaaatgctcaaatgagcatttcctttgagcatcatgtcggtattcaaaaagttttggattttggagcacttgattccaggagctcagcctgtatttagaaattaagcataacttctaaatagagctagctaatacttgctggttgcacttaagtatcatagtaattatcagcataaagtaaaaataagtatttactgcctaaaatgttgaaccaatgttttctgggaccatttctctaaatacacaaatggggagacatactagaaaaccttacaattaaatatgctggtagtgttagggttttagagcaaaacagaaatccaacccccaagaaagtcagggaaaagaagacaaaaatcagaagatgaacagctgcatatttctccacctaacactaggaggaaaaagtagaatatttgaaatacgatatggaatacaaatctgtgccatttagaacataatggtaggacgtagtaaacaagctacatcagcacaggacatggtttattgtcaaccatttaaacatataaacaaaactaagagtaagaaaataaaagacagatgctgtagcaaaagggcatttctctccaacatgattggccattattctccaaaatgtatggttaacagaaaattgaagaaaagtttgtatagagttattttaaatgattgatattttctggtttttttttttttttttttttttttttttgagacagggtcttgctctgtaatccaggctagagtgcaatggcatgatcacagctcattgcagccccaaacccccaggctcaaagtgatcctcctgcttcagcctcccgagtagctgggattaccaagcatgagccaccataccgagcaaatttaaaaaatttttttgtagagacagggtctctctatgttgctcaggctggttttgaactcctggactcaagcaatcctccctgcttcagcctcccaaagtgctgggattacaggcctccatgagcaaccacgcccagctcaagaatgattcacattttaattttcttttgaacaggtttaccactttgtatttgtgttttaggttttaagactaaatctgtgcaataatattccctagggattaaaagtaggggaaatacaaccctctccaaaagcagaaacaaaacttggggtggaaagaggaggtaaaaattacattcgcttttccaaatgagtctgaatcgtaaaaccataaagaatggttttactcattctttgtcagccatttgaaatcaataaactatgattcctacattttgtttgtattacacaaaaagtaaacaacaatgaaagctgtttttaaaagaataaaaaccaccaaccacaaatagaagagaaccccagacggttctcttggagggatgtttatcaccagtgccaaaagcctcccccctctgaaatgtttctctcagttgacaactttcaaatgatttaaagaacatgaagaacaagtagaacatgaagcttggatctgaatagtaaagaataatattggagtggtatttacaaaggagaggcagatatatgtgcctagcaccagatttttcaagtaagcaagttcagccccaaactaactgaagttttacatttttaaactctctccattatttcccagagttggaagctgtgaaatgtttcagcatggtgctattcactaatggtgtgaactcaaaaggtgggttttctgcagctgaactgattctaagtctcaggactccaagatacctccagtccaagtgtcgtggactctactggctttatacacctaatttgggactatccattttttccttctttaaagctggctagggaattccttcactaatgataatgtgtgcaaacacacacacatattgaaaatctataactaattctagcagccaaaagatgtttttccttaccagaaattacccaaagaaagttacattagaaataatatgactaaaaatatatttttaaagctatttaatactcatgatgtctaaactttcaatttattgtctgatttctggatatttctgtattttagattctacagacttcagattctgaagcttgttgaaaaagctaagttcctcaatatggatgaaaatctatctggctgtacttttagaggggaatttttctacttttgaaaaaaattctgaatatttatatatagtattaacagaataccccagtaagtcatatttcagataaatattctatagtataatttgcatcatacccaatattttagatattaaaataagggtaaaatttggaatataatcacttgtctgcatatttcccaatgtaagttttcatgtagaatattaaaatttaaattgatatttggatttataagctgttttccctgtatactatacgtatctattagcaatagagacaattttggagtcatggtatagtgaacctctctggctctccttgcacaaggctccatgagtcagtctgggcagtgcacgctacccttgcataactcactccccacactcaggcttaggggtactaacatgcaatcctaggacaacacttgacactagcactgacattttaaaattcattctcccaagtaataaaaaatatatatatagatagatatacacagagagatctgcagctgtactaattacttcaaatagcagcagacaaggaaaatacacgcttgcttgcttaagtttaaattcattttaagtttgctatattaaatttaaaaattaaaaaaatatcaacttactataaacaatttaaaatatgtataatacaacttcatggtcaaaacatttgaatagtctatgaaaacaggaaatacgttcatctgacatttctgtttagattccattcatgatttttcaatctgtctcttccaaaagaaaccataaagcagttgtcatattttatggcaactaattttgtttagggatttcctcatcacaaaaatactttatttcctattacaggggagttaaagaagaagaaaaaagaaatgagaaacaaagtggctttctccccacttgtcactattctcttcttcaaacattctgtacataagctgtctgagtcttttgaaccatttacaaattgtattttcaaaaattgaagaaaaaatatttagagtctaaaagtgttattttatacactgactatacaatatacattgaatgtttacacatacaaatacatcttaaagataaggttctccaaaggtttttcgacattccatcacccctgtacttggtggtctatcacagttgtgtgtactcttgacttgactaggtgtgagacgatcgtatgccatcttgtactctttatcaaaagcatctatatcaatgttttctcttcccagtgccacaagtgagagaaatagtatttctctgtataaactcctctgtcttttaaaatgtggacacttattcagtgtctctaaaatctgactcattggtccatagacatcattcattttaatgctttttaccatacttttcaacagttcctggttaaatgagttatcacttttttgcaataaatggaccattggatatttttgggtgtgtgcattccagagaatgtacaagggctgtcccggatcctgatgtaacttcatattgtcccataacatttgtattaaaacatatttgctatcttcagacatacagtggcggggaatctttgaatacttgttacagtgctcagaagaaagaatcaatccaggtaagttactgggcaagtcaagacgtctgaaataccataccaggttccaaaaaacaattggatgatggtccacaaagtctgctactgttattgcatgatcaccttcattttccaataagctttcaagttctttccataccactaaaggactaagatacggaacagtgacaggatcgggacttggaaggtgccattctaaacctaaagaatctgtagctccttgtaaagtagctggcaggctgcctgtagaaatgagcttctgtcttccagtatcttccttatccaaggggccagaagtactaatactcctggccattggaaatattggacatttagacatagctgtttttgatctattagcagggatctgaatacttcgggtgcaaaaattttcctgcagtttagatttgctatttagatcaaaattcccttgaacagagagagcagatgtgtcaagaccagaggctgatgttgaaatgcaagactgcctcgtctgacttgaaatggaggatggaaagtgcatattttctgttgatgggcttgactttagaaagtatcttccaggtcgtcttaaatctcttatttctatattcagaaagggtaagaagatattgccacagaatgggcatgtagtattgagatttgaatcatctgctgtccagccagccatgatttcctcatcatggacaagacaatcacaagttctacaccgagagcaacttgagatgagaacctccattgcatagttctggaagatatttgtattactcgcgttgaaggaagatgtcacttctgatttcccaggtaaggcaaacttcgacagagatccttccaaggatgcagaactttccaggcttattcggctgagatcaattctcttagtccctgaagtagcactggtctcttgagaggagataggtccttccaactcatggcagacatcttcatctgttaaagaggtagattcagaatcctgggctcccactgaagaaagactggtacgatcagaactttgatccttagatgatgtggtgtacatggtgaatcttgaataccatttgcttgctttctctgcaactccttttccagcagtgaacatactgtttcttagaacatctagtttaggtactagtagtgtatctaagttaaatgaaggtgatgagtgggttaatgtatcctgagattcttccctaaatgggcaagtaggtgagaaggctggagaagaccaaagtctatcccttggtttctcctcactttttgtgtaacttttagatttggtaagtctcactggcttaggagaattaggaggcagactagatcttctgcatgccttgaccaatggtggacttttcttatttaatttatcatcacatgcccgttgtaaatcaatgcttggtgtacgacttgtcaaaggactgctcatgttattcatatacatcacaatttcttcagctaaatcacgcctagcagatggtgttgaaatgcttttgctatcatcttcatcctcctcctcttcttctttttgctgctgttcagtctcagcaaccaaaagagagaggggatcaaatcctgttgcgacatcagttttttcaaaaggttttactgaaaagctgctgttcatacgttgaatcctcttgggattttgtgtagcaacacatcctgcttttgatacatctgtttcactgtctaagtcttctaagtcaaaaataacaggagaatccactttatctgccaaatagttagaaccatcaaaaggtgtatcatcatcactagattccttttctagactgtctctttttgatcttaaaggtggcttcccaatatcaagagtatttggtctcgtgctttttgagataacatttgaaagaatttttgcatcagctcccaatttttcaactatatctccaggggttgcttcctggttaattctattgagcataaatcccatcagtacccctccactaagattacggtttctatttccccagaccacttgctgctgcaaattagtttcattgtcacttttatgtcttttcctgaagcatctactttgaatgtttcgtgtttcatttgtatcttcaagagatgatattaagagcagctcaggtgtgctttccatgctttctcctgatattttaccagcactgttgttacttgtaccagtgaggcgaacgatactggaagaattttgataactgagcttaggaaggcaatcagcacttccttttgtactctcactctctgacaaggaactacaatcactcccttttttatctttttcttcttgaatgtcttcagtagatgtatcccctcttctaacttcatctttagataatgaattatatccaagatcagactggccacctgtactagatctatcatcagtagcatatactttgattaaacccgtattaaaaggtgcctgctccacagtgtgtgtcccatgaccactatccatgctgccatgactaacagcatccaggtcactgccatctgctgagagagttgtttgtgataagtgtgcatgcttctttaaagctcttttgaactgtgttactcctaaaacaacatttcttacttttgtccaaagaaaatagccactacgacttcttgaaggccaggtactttccaaaacagccttattataataaccataagtaatggcattggggtcaataccagctttctgcatttcaaaaagcactcgaactgcaagcactggctgatcatattgtccacagagttgcataagaatgcggtagcatacctcatcaggtggatccatcttctttgactgcatttttttaagcacatcatatgctgttttcagagccctgacttttgaatgacagactttcacataagctgggagacaaataaaccacagtccataacagtggcgcagtagacacctagaccacatctgagggatggaagagtacctctttgcaattttatgggctgatttaatttcctgttttgttcttctgaacatgggcaaagggctattaggactacttgattttgaaggcaatttgttcttctttgcttgtagaaatccttcaggtctttcaaataaattgttcctaagaactggaaatccattatagctgtactgtaaagggggttcttcaccattgggtaggtgggggatctcaggtggtgttacaaaaacagtgtgttcacttttgaaagattcatccagttctataagtcgtacttcaccgctcttgtccatatccactttatctacacaatcatcaaaaaatgccaggcttgcatctttgtcactaacaaaagaacattcttcaatgaagcgaataaacatttgtgttttggtcatcatgttatagaatttttgatgtgaccggtcccggcttcttaagaaagcttgtagggcaaagagagaggctgcatctgtggctgtctcagatggggcttgtgttattggccttaagtatgatctgtaaccttttaaaatagaggccatgaaaaacaaaaatgcctcttggatttccaaatctatcatgtgcaacctctttccagaattaaaatcatagtcatttattgctaaatccatgagtccatcatctctcggtctctgctgcaattttgccaattgctgatgcaaattattcagtgtgttcatcagatttttacatggcttctttggaagtatcttccaggctacatttttcttgtcaccaatttgagaaatagtgttggtatctacatcaacacaactgacatctggtggaggatcatagagatcaaagtatcttgaatcaatccctactatgaatggacatggtgcactcaagacatctgctaaagccagtgggcagagaggaacatacgggcatggccagtggaaagggaaaatcatagacactaatgcttctgtcacactagtaagcacggatggccgtagggaatggataagaattttatgttctgttactgcaaacaccagtagtgtcacagcattttcagggcctaaattctgcagtagtgttgaaaacttgccaccacttagtggaagaggtgaagacacaggctgactgagaatcagattatcatgtggtgataactgaactaaaatccgtggtctctgaggagatggaaaaggaactttatgcataaaatgagaaatatgcttctcaattggaaggacatgaggcccagagatggaataacgatacagaaaagtcagaaacttcctgaatgcatcaaaaaaaggccagtgagaaagaagacagatgcatttgttagtatgaattgttttggaactatcagacttcccatctgctgatgttaaacccaaaagaagtctctgcttttctgtgagattctcctcagagtatggttcataaaactgaatagcagcaccataaaccttttcagctgaggctccagttaaaacaaaagtagaaaatacaggcagagggtatttgctatttgatggccaacattcaatggttgcacccattggtaaacaaaatagaggaacagattccggtagtgagaatgactcataatcttcttgaggatatctacaaattaggccagctttgtaagatacagtgttcgtctttgccaccgattttttataacacaagtatactgctgatccccacatactgttattgagattcttgtcgactttgcagaacgtgtgtggtgggctttctcctttactgggtataataatacatatgtcagtgacagccaacgtattctgagtcatgttttcagaggctcttcggtaagtgatataaattctttgtgatgaggtactcccactaatatttgcggggcgcccatagggagtactctgaataatttcacaaccctgtttcaatctttctttccagtcatataaaacccccagatctgtaagtggaggcttatctcttcctcttctatagcaaaggtaaatctgtggccccacaagacttccattattaagatcagctgacaatccagttggggtaacatcaatacagatataatcctgtgggacttcctccccaagagatttgataataactgaaacatctgtaataggttcttttggtttagctactttatgacaagcatcattgaagtgaatttcttcttctagaggctttgaaacatcagttaatcctgctacaacaaagtagtcagcaacacgaggccccttgtcttcaatcatcttccattacagaaggttacatcacccagctggctcccgtgcgagcagcggatcgagctcggagagcggcgccggaatcccgcacgcgcggtagcggaacacgaggggctgaatgccgcggcgctctgagcccgcttagctcatccccagcccggcgctccgc

SEQ ID NO: 15515 - RNA, 10544 nt, Homo sapiens
  source 1..10544: mol_type = other RNA
gctgggattacaggcatgagccactgtacccagccaaaatggttactatatattttgaacattatattgcactgtcatcaatagattcgaaaatagttttaccaaattacaggcttagtcttttatagctgtctatatcaatattatttaaagattgagtaccaaagggggcaggaattggaatgtattatctagagcacagaatagtaaataatcaggaaaagggccgggcgcggtggctcatgcctataatcccagcactttgggaggccaaggtgggcggatcacgaggtcagtagatcgagaccatcctggctaacacggtgaaaccccgtctctactaaaaaaataccaaaaattagccgggcgaggtggcaggcgcctatagtcccagctactcgggaggctgaggcaggagaatggcgtgaaccccggggggcggagcctgcagtgagccgagatcgtgccactgcactccagcctgggcaacagcgagactccgtctcaaaaaaaaagaaaaaataaataatcaggaagaattggttggccttatgtgccaatgaatactcttggttctgacccttttttggtgggagggtcctccagcaggtgcagcttgcaatgtgtacggggactggatgctatgaaagatgtaatgagagggctcatgagcagagctgcctatccctgggggttcactaacgcctacaggacatcctggcccaagtctgcctgcacaactaaaggcacacttctggtctttaggtccttcgctgtatgagcaagcaaaacctggagaatttcacttgcagaaaatccaccagttgctgcaatagttttatcatagtactacatttgaaaaaaaaatatttaaatagtaaaggagggagccatccaaatgaacaggaactgtggaaaggcagcaataactttatcagaagaatctattaccatctcagagtacaagcacatgcgcagacttttgtaatcaaagatgaaaattcttcaatttgtgtactgctaattttgttaagaaatataagccagccaatatgcttactttgaggccaaaggagcaaggtagtatgaggatgttaagacaccaagtactaaggatattaaggtaaactggtatgcagctgctagagggttcagttttgaaataaagcttagtcttatatccagacaggaagaggcagcacatgctaactttagcacgaaggacaagggtcttctcaaagagacagcctgctctttctcttcttgctctgagataaagtgccaaatagcagctttcaagttctagtgagagaaataaaaataaagctgggctactgcacatcaccaaacaaataggtattttcatatcgcatattacaaagtagaggttgagtatcccttatcagaaatgtttcggaccagaagtgttttggatttcagatgtttttgaaatttggaatatttgaaaaatacaaactggttgaacatcccaaatatgaaatccaaaatgctcaaatgagcatttcctttgagcatcatgtcggtattcaaaaagttttggattttggagcacttgattccaggagctcagcctgtatttagaaattaagcataacttctaaatagagctagctaatacttgctggttgcacttaagtatcatagtaattatcagcataaagtaaaaataagtatttactgcctaaaatgttgaaccaatgttttctgggaccatttctctaaatacacaaatggggagacatactagaaaaccttacaattaaatatgctggtagtgttagggttttagagcaaaacagaaatccaacccccaagaaagtcagggaaaagaagacaaaaatcagaagatgaacagctgcatatttctccacctaacactaggaggaaaaagtagaatatttgaaatacgatatggaatacaaatctgtgccatttagaacataatggtaggacgtagtaaacaagctacatcagcacaggacatggtttattgtcaaccatttaaacatataaacaaaactaagagtaagaaaataaaagacagatgctgtagcaaaagggcatttctctccaacatgattggccattattctccaaaatgtatggttaacagaaaattgaagaaaagtttgtatagagttattttaaatgattgatattttctggtttttttttttttttttttttttttttttgagacagggtcttgctctgtaatccaggctagagtgcaatggcatgatcacagctcattgcagccccaaacccccaggctcaaagtgatcctcctgcttcagcctcccgagtagctgggattaccaagcatgagccaccataccgagcaaatttaaaaaatttttttgtagagacagggtctctctatgttgctcaggctggttttgaactcctggactcaagcaatcctccctgcttcagcctcccaaagtgctgggattacaggcctccatgagcaaccacgcccagctcaagaatgattcacattttaattttcttttgaacaggtttaccactttgtatttgtgttttaggttttaagactaaatctgtgcaataatattccctagggattaaaagtaggggaaatacaaccctctccaaaagcagaaacaaaacttggggtggaaagaggaggtaaaaattacattcgcttttccaaatgagtctgaatcgtaaaaccataaagaatggttttactcattctttgtcagccatttgaaatcaataaactatgattcctacattttgtttgtattacacaaaaagtaaacaacaatgaaagctgtttttaaaagaataaaaaccaccaaccacaaatagaagagaaccccagacggttctcttggagggatgtttatcaccagtgccaaaagcctcccccctctgaaatgtttctctcagttgacaactttcaaatgatttaaagaacatgaagaacaagtagaacatgaagcttggatctgaatagtaaagaataatattggagtggtatttacaaaggagaggcagatatatgtgcctagcaccagatttttcaagtaagcaagttcagccccaaactaactgaagttttacatttttaaactctctccattatttcccagagttggaagctgtgaaatgtttcagcatggtgctattcactaatggtgtgaactcaaaaggtgggttttctgcagctgaactgattctaagtctcaggactccaagatacctccagtccaagtgtcgtggactctactggctttatacacctaatttgggactatccattttttccttctttaaagctggctagggaattccttcactaatgataatgtgtgcaaacacacacacatattgaaaatctataactaattctagcagccaaaagatgtttttccttaccagaaattacccaaagaaagttacattagaaataatatgactaaaaatatatttttaaagctatttaatactcatgatgtctaaactttcaatttattgtctgatttctggatatttctgtattttagattctacagacttcagattctgaagcttgttgaaaaagctaagttcctcaatatggatgaaaatctatctggctgtacttttagaggggaatttttctacttttgaaaaaaattctgaatatttatatatagtattaacagaataccccagtaagtcatatttcagataaatattctatagtataatttgcatcatacccaatattttagatattaaaataagggtaaaatttggaatataatcacttgtctgcatatttcccaatgtaagttttcatgtagaatattaaaatttaaattgatatttggatttataagctgttttccctgtatactatacgtatctattagcaatagagacaattttggagtcatggtatagtgaacctctctggctctccttgcacaaggctccatgagtcagtctgggcagtgcacgctacccttgcataactcactccccacactcaggcttaggggtactaacatgcaatcctaggacaacacttgacactagcactgacattttaaaattcattctcccaagtaataaaaaatatatatatagatagatatacacagagagatctgcagctgtactaattacttcaaatagcagcagacaaggaaaatacacgcttgcttgcttaagtttaaattcattttaagtttgctatattaaatttaaaaattaaaaaaatatcaacttactataaacaatttaaaatatgtataatacaacttcatggtcaaaacatttgaatagtctatgaaaacaggaaatacgttcatctgacatttctgtttagattccattcatgatttttcaatctgtctcttccaaaagaaaccataaagcagttgtcatattttatggcaactaattttgtttagggatttcctcatcacaaaaatactttatttcctattacaggggagttaaagaagaagaaaaaagaaatgagaaacaaagtggctttctccccacttgtcactattctcttcttcaaacattctgtacataagctgtctgagtcttttgaaccatttacaaattgtattttcaaaaattgaagaaaaaatatttagagtctaaaagtgttattttatacactgactatacaatatacattgaatgtttacacatacaaatacatcttaaagataaggttctccaaaggtttttcgacattccatcacccctgtacttggtggtctatcacagttgtgtgtactcttgacttgactaggtgtgagacgatcgtatgccatcttgtactctttatcaaaagcatctatatcaatgttttctcttcccagtgccacaagtgagagaaatagtatttctctgtataaactcctctgtcttttaaaatgtggacacttattcagtgtctctaaaatctgactcattggtccatagacatcattcattttaatgctttttaccatacttttcaacagttcctggttaaatgagttatcacttttttgcaataaatggaccattggatatttttgggtgtgtgcattccagagaatgtacaagggctgtcccggatcctgatgtaacttcatattgtcccataacatttgtattaaaacatatttgctatcttcagacatacagtggcggggaatctttgaatacttgttacagtgctcagaagaaagaatcaatccaggtaagttactgggcaagtcaagacgtctgaaataccataccaggttccaaaaaacaattggatgatggtccacaaagtctgctactgttattgcatgatcaccttcattttccaataagctttcaagttctttccataccactaaaggactaagatacggaacagtgacaggatcgggacttggaaggtgccattctaaacctaaagaatctgtagctccttgtaaagtagctggcaggctgcctgtagaaatgagcttctgtcttccagtatcttccttatccaaggggccagaagtactaatactcctggccattggaaatattggacatttagacatagctgtttttgatctattagcagggatctgaatacttcgggtgcaaaaattttcctgcagtttagatttgctatttagatcaaaattcccttgaacagagagagcagatgtgtcaagaccagaggctgatgttgaaatgcaagactgcctcgtctgacttgaaatggaggatggaaagtgcatattttctgttgatgggcttgactttagaaagtatcttccaggtcgtcttaaatctcttatttctatattcagaaagggtaagaagatattgccacagaatgggcatgtagtattgagatttgaatcatctgctgtccagccagccatgatttcctcatcatggacaagacaatcacaagttctacaccgagagcaacttgagatgagaacctccattgcatagttctggaagatatttgtattactcgcgttgaaggaagatgtcacttctgatttcccaggtaaggcaaacttcgacagagatccttccaaggatgcagaactttccaggcttattcggctgagatcaattctcttagtccctgaagtagcactggtctcttgagaggagataggtccttccaactcatggcagacatcttcatctgttaaagaggtagattcagaatcctgggctcccactgaagaaagactggtacgatcagaactttgatccttagatgatgtggtgtacatggtgaatcttgaataccatttgcttgctttctctgcaactccttttccagcagtgaacatactgtttcttagaacatctagtttaggtactagtagtgtatctaagttaaatgaaggtgatgagtgggttaatgtatcctgagattcttccctaaatgggcaagtaggtgagaaggctggagaagaccaaagtctatcccttggtttctcctcactttttgtgtaacttttagatttggtaagtctcactggcttaggagaattaggaggcagactagatcttctgcatgccttgaccaatggtggacttttcttatttaatttatcatcacatgcccgttgtaaatcaatgcttggtgtacgacttgtcaaaggactgctcatgttattcatatacatcacaatttcttcagctaaatcacgcctagcagatggtgttgaaatgcttttgctatcatcttcatcctcctcctcttcttctttttgctgctgttcagtctcagcaaccaaaagagagaggggatcaaatcctgttgcgacatcagttttttcaaaaggttttactgaaaagctgctgttcatacgttgaatcctcttgggattttgtgtagcaacacatcctgcttttgatacatctgtttcactgtctaagtcttctaagtcaaaaataacaggagaatccactttatctgccaaatagttagaaccatcaaaaggtgtatcatcatcactagattccttttctagactgtctctttttgatcttaaaggtggcttcccaatatcaagagtatttggtctcgtgctttttgagataacatttgaaagaatttttgcatcagctcccaatttttcaactatatctccaggggttgcttcctggttaattctattgagcataaatcccatcagtacccctccactaagattacggtttctatttccccagaccacttgctgctgcaaattagtttcattgtcacttttatgtcttttcctgaagcatctactttgaatgtttcgtgtttcatttgtatcttcaagagatgatattaagagcagctcaggtgtgctttccatgctttctcctgatattttaccagcactgttgttacttgtaccagtgaggcgaacgatactggaagaattttgataactgagcttaggaaggcaatcagcacttccttttgtactctcactctctgacaaggaactacaatcactcccttttttatctttttcttcttgaatgtcttcagtagatgtatcccctcttctaacttcatctttagataatgaattatatccaagatcagactggccacctgtactagatctatcatcagtagcatatactttgattaaacccgtattaaaaggtgcctgctccacagtgtgtgtcccatgaccactatccatgctgccatgactaacagcatccaggtcactgccatctgctgagagagttgtttgtgataagtgtgcatgcttctttaaagctcttttgaactgtgttactcctaaaacaacatttcttacttttgtccaaagaaaatagccactacgacttcttgaaggccaggtactttccaaaacagccttattataataaccataagtaatggcattggggtcaataccagctttctgcatttcaaaaagcactcgaactgcaagcactggctgatcatattgtccacagagttgcataagaatgcggtagcatacctcatcaggtggatccatcttctttgactgcatttttttaagcacatcatatgctgttttcagagccctgacttttgaatgacagactttcacataagctgggagacaaataaaccacagtccataacagtggcgcagtagacacctagaccacatctgagggatggaagagtacctctttgcaattttatgggctgatttaatttcctgttttgttcttctgaacatgggcaaagggctattaggactacttgattttgaaggcaatttgttcttctttgcttgtagaaatccttcaggtctttcaaataaattgttcctaagaactggaaatccattatagctgtactgtaaagggggttcttcaccattgggtaggtgggggatctcaggtggtgttacaaaaacagtgtgttcacttttgaaagattcatccagttctataagtcgtacttcaccgctcttgtccatatccactttatctacacaatcatcaaaaaatgccaggcttgcatctttgtcactaacaaaagaacattcttcaatgaagcgaataaacatttgtgttttggtcatcatgttatagaatttttgatgtgaccggtcccggcttcttaagaaagcttgtagggcaaagagagaggctgcatctgtggctgtctcagatggggcttgtgttattggccttaagtatgatctgtaaccttttaaaatagaggccatgaaaaacaaaaatgcctcttggatttccaaatctatcatgtgcaacctctttccagaattaaaatcatagtcatttattgctaaatccatgagtccatcatctctcggtctctgctgcaattttgccaattgctgatgcaaattattcagtgtgttcatcagatttttacatggcttctttggaagtatcttccaggctacatttttcttgtcaccaatttgagaaatagtgttggtatctacatcaacacaactgacatctggtggaggatcatagagatcaaagtatcttgaatcaatccctactatgaatggacatggtgcactcaagacatctgctaaagccagtgggcagagaggaacatacgggcatggccagtggaaagggaaaatcatagacactaatgcttctgtcacactagtaagcacggatggccgtagggaatggataagaattttatgttctgttactgcaaacaccagtagtgtcacagcattttcagggcctaaattctgcagtagtgttgaaaacttgccaccacttagtggaagaggtgaagacacaggctgactgagaatcagattatcatgtggtgataactgaactaaaatccgtggtctctgaggagatggaaaaggaactttatgcataaaatgagaaatatgcttctcaattggaaggacatgaggcccagagatggaataacgatacagaaaagtcagaaacttcctgaatgcatcaaaaaaaggccagtgagaaagaagacagatgcatttgttagtatgaattgttttggaactatcagacttcccatctgctgatgttaaacccaaaagaagtctctgcttttctgtgagattctcctcagagtatggttcataaaactgaatagcagcaccataaaccttttcagctgaggctccagttaaaacaaaagtagaaaatacaggcagagggtatttgctatttgatggccaacattcaatggttgcacccattggtaaacaaaatagaggaacagattccggtagtgagaatgactcataatcttcttgaggatatctacaaattaggccagctttgtaagatacagtgttcgtctttgccaccgattttttataacacaagtatactgctgatccccacatactgttattgagattcttgtcgactttgcagaacgtgtgtggtgggctttctcctttactgggtataataatacatatgtcagtgacagccaacgtattctgagtcatgttttcagaggctcttcggtaagtgatataaattctttgtgatgaggtactcccactaatatttgcggggcgcccatagggagtactctgaataatttcacaaccctgtttcaatctttctttccagtcatataaaacccccagatctgtaagtggaggcttatctcttcctcttctatagcaaaggtaaatctgtggccccacaagacttccattattaagatcagctgacaatccagttggggtaacatcaatacagatataatcctgtgggacttcctccccaagagatttgataataactgaaacatctgtaataggttcttttggtttagctactttatgacaagcatcattgaagtgaatttcttcttctagaggctttgaaacatcagttaatcctgctacaacaaagtagtcagcaacacgaggccccttgtcttcaatcatcttccattacagaaggttacattatatatataaaaatactaaatcctcagcagtcttttgataaaggcagccgataaactttgcttaactcaggatttcccaagc

SEQ ID NO: 15516 - RNA, 9159 nt, Homo sapiens
  source 1..9159: mol_type = other RNA
gctgggattacaggcatgagccactgtacccagccaaaatggttactatatattttgaacattatattgcactgtcatcaatagattcgaaaatagttttaccaaattacaggcttagtcttttatagctgtctatatcaatattatttaaagattgagtaccaaagggggcaggaattggaatgtattatctagagcacagaatagtaaataatcaggaaaagggccgggcgcggtggctcatgcctataatcccagcactttgggaggccaaggtgggcggatcacgaggtcagtagatcgagaccatcctggctaacacggtgaaaccccgtctctactaaaaaaataccaaaaattagccgggcgaggtggcaggcgcctatagtcccagctactcgggaggctgaggcaggagaatggcgtgaaccccggggggcggagcctgcagtgagccgagatcgtgccactgcactccagcctgggcaacagcgagactccgtctcaaaaaaaaagaaaaaataaataatcaggaagaattggttggccttatgtgccaatgaatactcttggttctgacccttttttggtgggagggtcctccagcaggtgcagcttgcaatgtgtacggggactggatgctatgaaagatgtaatgagagggctcatgagcagagctgcctatccctgggggttcactaacgcctacaggacatcctggcccaagtctgcctgcacaactaaaggcacacttctggtctttaggtccttcgctgtatgagcaagcaaaacctggagaatttcacttgcagaaaatccaccagttgctgcaatagttttatcatagtactacatttgaaaaaaaaatatttaaatagtaaaggagggagccatccaaatgaacaggaactgtggaaaggcagcaataactttatcagaagaatctattaccatctcagagtacaagcacatgcgcagacttttgtaatcaaagatgaaaattcttcaatttgtgtactgctaattttgttaagaaatataagccagccaatatgcttactttgaggccaaaggagcaaggtagtatgaggatgttaagacaccaagtactaaggatattaaggtaaactggtatgcagctgctagagggttcagttttgaaataaagcttagtcttatatccagacaggaagaggcagcacatgctaactttagcacgaaggacaagggtcttctcaaagagacagcctgctctttctcttcttgctctgagataaagtgccaaatagcagctttcaagttctagtgagagaaataaaaataaagctgggctactgcacatcaccaaacaaataggtattttcatatcgcatattacaaagtagaggttgagtatcccttatcagaaatgtttcggaccagaagtgttttggatttcagatgtttttgaaatttggaatatttgaaaaatacaaactggttgaacatcccaaatatgaaatccaaaatgctcaaatgagcatttcctttgagcatcatgtcggtattcaaaaagttttggattttggagcacttgattccaggagctcagcctgtatttagaaattaagcataacttctaaatagagctagctaatacttgctggttgcacttaagtatcatagtaattatcagcataaagtaaaaataagtatttactgcctaaaatgttgaaccaatgttttctgggaccatttctctaaatacacaaatggggagacatactagaaaaccttacaattaaatatgctggtagtgttagggttttagagcaaaacagaaatccaacccccaagaaagtcagggaaaagaagacaaaaatcagaagatgaacagctgcatatttctccacctaacactaggaggaaaaagtagaatatttgaaatacgatatggaatacaaatctgtgccatttagaacataatggtaggacgtagtaaacaagctacatcagcacaggacatggtttattgtcaaccatttaaacatataaacaaaactaagagtaagaaaataaaagacagatgctgtagcaaaagggcatttctctccaacatgattggccattattctccaaaatgtatggttaacagaaaattgaagaaaagtttgtatagagttattttaaatgattgatattttctggtttttttttttttttttttttttttttttgagacagggtcttgctctgtaatccaggctagagtgcaatggcatgatcacagctcattgcagccccaaacccccaggctcaaagtgatcctcctgcttcagcctcccgagtagctgggattaccaagcatgagccaccataccgagcaaatttaaaaaatttttttgtagagacagggtctctctatgttgctcaggctggttttgaactcctggactcaagcaatcctccctgcttcagcctcccaaagtgctgggattacaggcctccatgagcaaccacgcccagctcaagaatgattcacattttaattttcttttgaacaggtttaccactttgtatttgtgttttaggttttaagactaaatctgtgcaataatattccctagggattaaaagtaggggaaatacaaccctctccaaaagcagaaacaaaacttggggtggaaagaggaggtaaaaattacattcgcttttccaaatgagtctgaatcgtaaaaccataaagaatggttttactcattctttgtcagccatttgaaatcaataaactatgattcctacattttgtttgtattacacaaaaagtaaacaacaatgaaagctgtttttaaaagaataaaaaccaccaaccacaaatagaagagaaccccagacggttctcttggagggatgtttatcaccagtgccaaaagcctcccccctctgaaatgtttctctcagttgacaactttcaaatgatttaaagaacatgaagaacaagtagaacatgaagcttggatctgaatagtaaagaataatattggagtggtatttacaaaggagaggcagatatatgtgcctagcaccagatttttcaagtaagcaagttcagccccaaactaactgaagttttacatttttaaactctctccattatttcccagagttggaagctgtgaaatgtttcagcatggtgctattcactaatggtgtgaactcaaaaggtgggttttctgcagctgaactgattctaagtctcaggactccaagatacctccagtccaagtgtcgtggactctactggctttatacacctaatttgggactatccattttttccttctttaaagctggctagggaattccttcactaatgataatgtgtgcaaacacacacacatattgaaaatctataactaattctagcagccaaaagatgtttttccttaccagaaattacccaaagaaagttacattagaaataatatgactaaaaatatatttttaaagctatttaatactcatgatgtctaaactttcaatttattgtctgatttctggatatttctgtattttagattctacagacttcagattctgaagcttgttgaaaaagctaagttcctcaatatggatgaaaatctatctggctgtacttttagaggggaatttttctacttttgaaaaaaattctgaatatttatatatagtattaacagaataccccagtaagtcatatttcagataaatattctatagtataatttgcatcatacccaatattttagatattaaaataagggtaaaatttggaatataatcacttgtctgcatatttcccaatgtaagttttcatgtagaatattaaaatttaaattgatatttggatttataagctgttttccctgtatactatacgtatctattagcaatagagacaattttggagtcatggtatagtgaacctctctggctctccttgcacaaggctccatgagtcagtctgggcagtgcacgctacccttgcataactcactccccacactcaggcttaggggtactaacatgcaatcctaggacaacacttgacactagcactgacattttaaaattcattctcccaagtaataaaaaatatatatatagatagatatacacagagagatctgcagctgtactaattacttcaaatagcagcagacaaggaaaatacacgcttgcttgcttaagtttaaattcattttaagtttgctatattaaatttaaaaattaaaaaaatatcaacttactataaacaatttaaaatatgtataatacaacttcatggtcaaaacatttgaatagtctatgaaaacaggaaatacgttcatctgacatttctgtttagattccattcatgatttttcaatctgtctcttccaaaagaaaccataaagcagttgtcatattttatggcaactaattttgtttagggatttcctcatcacaaaaatactttatttcctattacaggggagttaaagaagaagaaaaaagaaatgagaaacaaagtggctttctccccacttgtcactattctcttcttcaaacattctgtacataagctgtctgagtcttttgaaccatttacaaattgtattttcaaaaattgaagaaaaaatatttagagtctaaaagtgttattttatacactgactatacaatatacattgaatgtttacacatacaaatacatcttaaagataaggttctccaaaggtttttcgacattccatcacccctgtacttggtggtctatcacagttgtgtgtactcttgacttgactaggtgtgagacgatcgtatgccatcttgtactctttatcaaaagcatctatatcaatgttttctcttcccagtgccacaagtgagagaaatagtatttctctgtataaactcctctgtcttttaaaatgtggacacttattcagtgtctctaaaatctgactcattggtccatagacatcattcattttaatgctttttaccatacttttcaacagttcctggttaaatgagttatcacttttttgcaataaatggaccattggatatttttgggtgtgtgcattccagagaatgtacaagggctgtcccggatcctgatgtaacttcatattgtcccataacatttgtattaaaacatatttgctatcttcagacatacagtggcggggaatctttgaatacttgttacagtgctcagaagaaagaatcaatccaggtaagttactgggcaagtcaagacgtctgaaataccataccaggttccaaaaaacaattggatgatggtccacaaagtctgctactgttattgcatgatcaccttcattttccaataagctttcaagttctttccataccactaaaggactaagatacggaacagtgacaggatcgggacttggaaggtgccattctaaacctaaagaatctgtagctccttgtaaagtagctggcaggctgcctgtagaaatgagcttctgtcttccagtatcttccttatccaaggggccagaagtactaatactcctggccattggaaatattggacatttagacatagctgtttttgatctattagcagggatctgaatacttcgggtgcaaaaattttcctgcagtttagatttgctatttagatcaaaattcccttgaacagagagagcagatgtgtcaagaccagaggctgatgttgaaatgcaagactgcctcgtctgacttgaaatggaggatggaaagtgcatattttctgttgatgggcttgactttagaaagtatcttccaggtcgtcttaaatctcttatttctatattcagaaagggtaagaagatattgccacagaatgggcatgtagtattgagatttgaatcatctgctgtccagccagccatgatttcctcatcatggacaagacaatcacaagttctacaccgagagcaacttgagatgagaacctccattgcatagttctggaagatatttgtattactcgcgttgaaggaagatgtcacttctgatttcccaggtaaggcaaacttcgacagagatccttccaaggatgcagaactttccaggcttattcggctgagatcaattctcttagtccctgaagtagcactggtctcttgagaggagataggtccttccaactcatggcagacatcttcatctgttaaagaggtagattcagaatcctgggctcccactgaagaaagactggtacgatcagaactttgatccttagatgatgtggtgtacatggtgaatcttgaataccatttgcttgctttctctgcaactccttttccagcagtgaacatactgtttcttagaacatctagtttaggtactagtagtgtatctaagttaaatgaaggtgatgagtgggttaatgtatcctgagattcttccctaaatgggcaagtaggtgagaaggctggagaagaccaaagtctatcccttggtttctcctcactttttgtgtaacttttagatttggtaagtctcactggcttaggagaattaggaggcagactagatcttctgcatgccttgaccaatggtggacttttcttatttaatttatcatcacatgcccgttgtaaatcaatgcttggtgtacgacttgtcaaaggactgctcatgttattcatatacatcacaatttcttcagctaaatcacgcctagcagatggtgttgaaatgcttttgctatcatcttcatcctcctcctcttcttctttttgctgctgttcagtctcagcaaccaaaagagagaggggatcaaatcctgttgcgacatcagttttttcaaaaggttttactgaaaagctgctgttcatacgttgaatcctcttgggattttgtgtagcaacacatcctgcttttgatacatctgtttcactgtctaagtcttctaagtcaaaaataacaggagaatccactttatctgccaaatagttagaaccatcaaaaggtgtatcatcatcactagattccttttctagactgtctctttttgatcttaaaggtggcttcccaatatcaagagtatttggtctcgtgctttttgagataacatttgaaagaatttttgcatcagctcccaatttttcaactatatctccaggggttgcttcctggttaattctattgagcataaatcccatcagtacccctccactaagattacggtttctatttccccagaccacttgctgctgcaaattagtttcattgtcacttttatgtcttttcctgaagcatctactttgaatgtttcgtgtttcatttgtatcttcaagagatgatattaagagcagctcaggtgtgctttccatgctttctcctgatattttaccagcactgttgttacttgtaccagtgaggcgaacgatactggaagaattttgataactgagcttaggaaggcaatcagcacttccttttgtactctcactctctgacaaggaactacaatcactcccttttttatctttttcttcttgaatgtcttcagtagatgtatcccctcttctaacttcatctttagataatgaattatatccaagatcagactggccacctgtactagatctatcatcagtagcatatactttgattaaacccgtattaaaaggtgcctgctccacagtgtgtgtcccatgaccactatccatgctgccatgactaacagcatccaggtcactgccatctgctgagagagttgtttgtgataagtgtgcatgcttctttaaagctcttttgaactgtgttactcctaaaacaacatttcttacttttgtccaaagaaaatagccactacgacttcttgaaggccaggtactttccaaaacagccttattataataaccataagtaatggcattggggtcaataccagctttctgcatttcaaaaagcactcgaactgcaagcactggctgatcatattgtccacagagttgcataagaatgcggtagcatacctcatcaggtggatccatcttctttgactgcatttttttaagcacatcatatgctgttttcagagccctgacttttgaatgacagactttcacataagctgggagacaaataaaccacagtccataacagtggcgcagtagacacctagaccacatctgagggatggaagagtacctctttgcaattttatgggctgatttaatttcctgttttgttcttctgaacatgggcaaagggctattaggactacttgattttgaaggcaatttgttcttctttgcttgtagaaatccttcaggtctttcaaataaattgttcctaagaactggaaatccattatagctgtactgtaaagggggttcttcaccattgggtaggtgggggatctcaggtggtgttacaaaaacagtgtgttcacttttgaaagattcatccagttctataagtcgtacttcaccgctcttgtccatatccactttatctacacaatcatcaaaaaatgccaggcttgcatctttgtcactaacaaaagaacattcttcaatgaagcgaataaacatttgtgttttggtcatcatgttatagaatttttgatgtgaccggtcccggcttcttaagaaagcttgtagggcaaagagagaggctgcatctgtggctgtctcagatggggcttgtgttattggccttaagtatgatctgtaaccttttaaaatagaggccatgaaaaacaaaaatgcctcttggatttccaaatctatcatgtgcaacctctttccagaattaaaatcatagtcatttattgctaaatccatgagtccatcatctctcggtctctgctgcaattttgccaattgctgatgcaaattattcagtgtgttcatcagatttttacatggcttctttggaagtatcttccaggctacatttttcttgtcaccaattttgggatttgtttttctttcaaacttcaggctggggcttcagaaattctaattgaaggaaagtagaaagctgtcagttcgctagtctagtcctccaccggtttgggagggtggtaatggcaagaattcatgagcacaaacaacttatctttctttgattctttaactcattagtgatcaaagcagaaagaaaagagctcagacctca

SEQ ID NO: 15517 - RNA, 29686 nt, Homo sapiens
  source 1..29686: mol_type = other RNA
gctgggattacaggcatgagccactgtacccggccccacaatttttttttttttttttttttggagagatgggatcttgctatgttgatcaggctggaaacctgggtcttgaataatggatacatttggaagtgcagagcaaaggccagagagatatccaagccagagagatatccaaggcagaacaaagctcataatttaacaagaaaggtaggcatagataggcctaattatgatgaatgctctcttaccagtataaacaaattacaaagggagtgatgagaagaggcaatgaagtttggggagggaaagaaaagtctgtggtggaggtgataacctgaacttggctttgaggaataaagagttttatatcagggcatcaagagaaggatattcaaggtacttaggaccagaacaggcaaaggcactgaagcaagagagtctggggcaagaatgtctctattgggtcaagactttgacaatattaaagattccattttcttcatatatgcccccctgctgtctttccaataaaggtaagccctgaagcctgacagtcacaggaaaggagagggtgtgtactagagtaacagcacagttgctactcagctgtgaatctcagagcctgcctttattatcttgattattctttggcatctctaggaagatgataagtagtcttcaaagtcagactttactgagaatgagaagggagttctacatgctaagagctccattcacatactaaaagcaaagcttggacaactgaacatgagttttactcctaaccatggataagagaaactgagaatacgatgtgagaagagtctcttcattaggcaggagtggaatgactcccagggcagggagagattgattgagattgcaattgccctgttgggaaataaacggaaacttcaggatgggtatgcgagtcttggagcagcagggttagtcaactactttcctggcatagcctggggaagactgcaagccactcaaaaaagtcctactcatgacttagaggcttacccagtatggcacaggagcactagctcagcattggtggaaggaggtgtctagtcagtctgagaaaatgttggcttcccaaagcttgagcaagatgttcagtacatcccaaagttccaacatcatcccttcccacccactccaaagcccagcagattaacagtcccatagttgggacatggaagctattaaggtagagaccttgagaccaaaggcaatgacagagttgtggtcaggagcagggcatgacagcagtgaacaaaagccagggacccacttacattacccagtagactcagtgacatccagcaaagatggcaggatgagcaccagcagcaggaccgtcaaggacctcagcacatacattagagaaactctttcctgtgtcacctggagatgactgttctcacccactagatgccatcatgaggaagaagctaggaagaacctttgaaaagctgagcatttatccaaagagatggttttaagcctgagataggctatttgaatcgaaagagaacgttatctttgattggcaagtttaaggccatccacctcgtcccacaccttcccaaaaccagatgggatgcatgagaaattgatgtgaaatgaaggaactgtaacttcttttctgcatgatctgagttttaatgtgtgggagctgggaagagggaagaacattgatagaaaatctgaaagcccacagggaatgtggtctaaagcagaggtttaagtcctggctgataatcattttgggttttctgaaaatgcagatcccagtgctccaattccagacctgctaaagcagaatctcacaattgaggccagggaacctacattttagaagctctccttctgactccaatttggaaaccatttatttaaccactagtacaaaaactggccttgaataagacatcacttcctccaagtctgagtacagcacgcaagggcaactgcagcaaatggaggggtgatttagtaaggagggggtgaaaccgaaaatcaacaaggtttgtgtgaactggtctcgacacacttggctgtgaatagcagggatagaaagtagttatggggcttgcaaggacattgtcttaattttcctgttgtcttaacagaggatttactgagcccatgtatgctgtaggaaaaagctagtggtgccagagtttaagttttcagaggaggaataattgacctatgtatgagttctagagaagccttgcagacttacccagggctcagagcacatggcttagtcctgacataaaataccatttttcctctaccacttggctaagaagctgaggaggaactggcagtgagggaggaggttgagaatgaaagttctggagagtcacctaagagacggtaaacacatacctcatgtcttggcttctagagcccggagataagatcagcttcccttgaaaatgttagctcccatgccacatttagtcaagacaacaataacaaaaggctttcttcagggagggcagtggaagtgagtttgagataaaaaggaatttatttatttgcacctatgtattgttcagaagttttaggtcttatgaaaaaaagatttttataaattatacacaattgggtagctttaaaaaataccaaaatatacagtggtcaccctaaaactaacatttttggataatacacttataaattggaaaatgagaaaagatagtctggtataactgcctgaacaacttattaagaacattaacaagtaataacacatattttaatgtaatattgctgactaatttggcacatttaatacacgtccaatatattttctatgtactgtgaaagcttttgggaaaataaagcagcttgtgttacaaaaactgcaacctttcacaaaggttacccacaaaatacttttgcctagccactgcctgtccaacttcagagtggcaccacccttgctattgatctttgtaaccaacgacaattatttcaaaacaattatacaaccctcatttttctttaaaatctttgtcttcctttacttccctgaatacacacgtagtttaccatgacatgggtcttttttttttttttttggagacgtagttttgcactgtcgcccaggctggagtgcagtggcacatctaggctcactgcaacctccacttctcaggttcaagccaatcttctgcctcagcctcccaagtagcgggatcataggcacccaccaatacacccatctaattttttgtatttttagtagagagggggtttcactatgttggccaggctggtctcaaactcctgacctcgtgatcggcccacctcagcctcccaaagtgctgggattacaggcataagccaccgcgcacggcccatgacatgcgtatttctacagcaatgctgtattcccaaatagagttttcttttagagagcctctctctgtgttgacataaatggtgttcagcagtagaacctgaagtaggacacatttcagagagaagtggtgatctcagaatcagtatgcagtactcacaggagccctttgggctctccgcttacatagcttgtctgttctgccccagtgagtcttttctcaggcagagcctcccacttttggcagaggctttttgacttgactttggatttgtcttggttctaagaccactttaataaaggactttacatccctcctgggatgacaaaagactttttgtctttcctggcaagtcctttttgatataaagacaagtgtccctctggtttgagtactctggatttaaaaacaatttttttttagagacagtgtctcactatactgctgaggctggtcttgaactcatgggctcaagcgatcctcctgccttggcctcccaaagtgctgggattacaggcatgggccactgcgcctggctgagtactctggattctgaggcatgccttttctggtaaatttactttgggttcttctgtgtttatattattttttaatctgcatgactgggttaacacttttgggaacactgattttggtttcgtttcgatatggttacatgcatctgtaaatgatttggctcttttcccctgtttctgaacatctcccaagagcaaaaataaacattctaaattttgggcacaggatggctcttttaaagccactagggcaatcgccaccagttaaaacactggtccaaacacctgacttatctgtcaggatttacagaattttctttgctcttaagagattgagaagaaacaaaatggaaattctcaaacattaaggcatgcctgcttttctgggacttcaggtcagctatgtggcttttcctcatgcatgtttttggatcaatgaccatcatagagattgtctatgctttgtctaaactccccaagcttttttattcttagtaccaagagactgcagctatagagttgatatgtagagtcttctaagctctctaattttttttctgcctactttaaatctgctgtttctgccagtgttgagatgaaactcactccttacggcattccagccaagaacaaaaagaaaaaaaaaggtcttaaagggccttaaattaatggctttataaattataatagttccctggcaaccaacacctagaattaagaagtatcccttttaatgtaaatttaggtttgcctaataactgcttagggtgatggaacagttaattaaaggattaatagcctaaaagaactagataaatacgtataaaaattaggctctcaaacaggtcaaaatcttgagctcagggcaataatataaggtatctctggtatagcataaaaattgcttgcctgctatgcaaaggctaaaagaacaaaacaaaaacccctcatccacaactgctaaaatgcttccctgcctgcactgactagtcaaaaaaaccagaatggcaaacaaaagatttgttactaaaaattcaaggccacctggagattgttttttcttatacaattcagccagtcctagctaaaaatgtaagcatttaaatattaacattaaactcatttgaaactgaaaaaagggaaaaaaggggttggggaggtggggtaagaggttttttaaaaatccaaactgctatttaccaaaacttttggttcacagctttcataagattacctattctgcatgtttacccagctgagcaggtcccactttctcagaaatataatttgaatccaataactgtcttttataaaccagcaagcctgtattactatcgtatgactaaaattctaaaatgaaagctatgtttgtgtatgtgtatgtttaggtgtgtttacacatatgtatatatatgttgtatgttgtgtctacgtggtaaaatctggcagttggccacaaatcccttaaggaattctattcatcaaataaatgagtgctaatacaaaatatatagtaattaacacaagtgccttttagttaatataacttaaacatctgataagctggttttaaaataattggtaaatcaaaaataagtgtctttaaaatttttgcctgaatttactactcagttttatatttgtctctgttagactttttaaggtcataaaactataaactcaacttaaaaacagaatgatctttgtataactgtaagttgaactaattttgtattattgacttcagctgtgtcctctgagttactggcaaaatacctacatatttcatttttatggttcttaattgaacacatgatactcacaggtaataaaaatggttaacaggaaaataacttgaaatgactagctatgtctaatatctcagtttttataagtaatctaggaataattgttaaaaatgaattgggggccaggtgcagtggctcacgcctgtaatcctagcactttgggaggccaaggcgggcagatcacgaggtcaggagatcgagatcacggtgaaacctcgtctctactaaaaatacaaaaaattggctgggcgcggtggcgggcgcctgtagtcccagctactcgggaggctgaggcaggagaatggcatgaacccagaaggcggagcttgcagtgagccgagatcacgccactgcactccagcctgggtgacagagcgagactccgtctcaaaaaaaaaaaaaaaaaaaagaattggatggattataaacgggataagcaagggtgagacatggtggtatgcaggtatgcatctatagttccagctactcaggaaacggaggcaggaggattgtgtgagttggagtttgaggctgcagtgtgctacaattgtgcctgtgaacagccactgaactccagcctgggtaacacagcaagacattgtctctaaaaaataaaccaaaagaatgtttttaaaaataggatgttaatgaacttttcatgtaatttgaaatcttataaattaatcttcagtaaatgtctggatcatttccaaaaaaaaacaataaactgctgaaaatattagtttgttcttggcttcctaaattatagaaagactaaatatatttgggcctattaatatacaaagttataaggaaacatgtttctaaaaattataatatggttctcatttataaaatgctgatataacacttcaaaattttgcttcctaggttttcactaaaaattaaggttaataagttaaaatttgaaaatacacaattccatatacaaagtgtacccaaaaaaagatgttttgatgagaaaagttataaggcataaaaattgctttttattgggaaaaaagttgtttaaattcagagtttattagaggttgtttcaaatatggaaacaagacagaaaggaaccactaagtaggaggaggagagaaatatgaaggaagttaatgggtgtgagaatgtacctttggtaaggaaggttacaaaattaacagaataattctgtatgagtcttgcatagtaactttttatcctaaagcaggatgaccagttgtttaaggggaagtataaaacaaagcagaaagtttaagcatgtcactgaaggtctgtgcagatcatgaaatgttcatgaaggatacatttatgaaaggagttgtgtgtaatgaagttggcaataggtcagaatgaaatcataagacattgagcttacatatatacttgtacatatgtatatgtacaataatacagtatattctatacatatgctatatatttgtatatacacgatagtgtaaatgctatacatgcactatacacacacacacacacacacacacacacacacacacacacacacaaaatttggtccccaatgttagaacaaggttctttttaaggatctggtcttaataaaattgaaagaggttttaatttttaattctaaaatcagccatcttctaaaccacagtttaaatttctgccatatttccttctgagatccgtttaatttcccctagattcaggttagaaaggctgtcttttttcatttaagatggtcatttcatttcttgaggtagagttttcttcttgaagatcctgatttatatctcacaagttcaacctttgctgtatcttgctgcaccttatttgtaggtcacacatcattgcctttagctctttctccccttaagaaggtacatctttttgtttggcaggggtgataactcttaactttttcattagctcctgtaacttttttcctctggttctaactcttgctgttataacttgatactgaaatgttctgtagaaggcctagaaaagcaatgttttcctccagtataacttgattctgaattcttggctcttctcatgtttgaattgttccacgcaagcaggaaatttctcgtaatttttccaagagccatgtattctgttcaacatactagctttcttatttacattcctctataaggcgtacactcataaccttggaaatactcttcctgtgtctgattaaattcaagtaccttttcatcagattcaactttcagtatatccaaataggcttcccataagtaaaggcagtcacactgcaagagatttttctttaccattttggcaactggcctaagaaaaattttatgttctatcaagataaattcttgtgtttaagttttttttttgcttgggaaaaatgaagctttgaaaagatggtttttaaatgtatgtaactttctgcattgcttcttaagtcttttgattatcattcttgttaaatattttatagtgacctgtgatcctgtttcgaacttttgacatctttgacaggcttctctaggctcaagttctaaattaagtgtttttgacttaaaattacctttgagttttccacttgggcctctggaaagcctcagagcatgtgtatgccatctggtagagatgttagctaattaggcttctttgatgtattaaattgtatgaaaagcattgtctaatgatgtaatactagacacagttacatttatgagtatgttattgatatgagtgttccaaaattgtacgatgccgttagaaatatgtcatcagtcataattctgattatgctgtttgccacaaaaataaccaaaactctttgtctatttctggttatggtaaactctcatcagatttttaatcatggttattctaagtttttgtaattcccagttattgctttttctctaaaagcatttgcaatcagattcatggaaaagatgctaacacacttttaaatacaggttactaatcactttaataccaatggactaaatattttttcagaacttcaagaaactgatgagtccatgtaactactaattaagatcaaccacaacaaaaaaagttacatgagactaagtaactgaagatgtgtctgtgacttttatttgaagcattattgtttttttacttaaatgttttgttttccatatttaaagaaattctctcatgctatctatagtttacagcaatttggaatacttttgtgaacaaaggtagaaatatttgcttttcctttcttcttgatccctccaatttggaaactattttgagtattcatttgtttttgtttttgagacggagtctcgctctgttgccccagctggaatgcagtggcacgatcttgtttcagtgcaacttctgcctccagggttcaagcaattctgtctcagcctcccaagtagctgggactacaggcatgcaccaccacacccagctaatttttgtattttttagtagagacggtggccggggggaggtttcactatgttggccaggctggtttcaaactcctgacctcaggtgttccacctgtcttggcctcccaaagagctgggattacaggcatgagccactgtgcccagcctatttgtgagtactcttaaggcaatatgatttgcctaagttcaataaaaatcggctctcgttataacaggatacaattggaaacactggttgtattaccaaggctttgattaaaatgtcatatttgagaatgtgtagaatgcctggcttcaatggttctcagcattacactgaattaaaaattatcatttcctggcaggcccaggaaccttaaaactataggtaaaatctaaagtctaccttgacttagcttcttagcctcaaggaggtttttaaatctgagattactgtgaccatactactattcttgcagacaaaatctgataaagtttacaaatctgttttattctgaacatctttggtaaaaatcagggtaactttaagtttctgaagaaagctatatgtacctgttattagatcacagctctgtaccgttttgaaactcctgttatccacctgcagactggatttgctcctgaatcctcctaatttccttcaatatttggctatgactctctaagaaaaaaaactactcccatgctctgaggcctataagctaagatgtgattaatttttaaaggagcaagtctcatgctgatgtatgggtcacacaaaagttcaccataccaaccaatgccatagctagagacattcaaactgcaaaccaggacaaaaagttgatgatttcaggctgtagacatttttcctaagacatcagagcaagaattgtattacaatttgatttattcaattggttgcctgtaagcctaggttcagggctcaaaaccattatgcaaactgggattgtcacattactattaattttgtgtatttcctttttaaactttgtatctgttatttgccaaattttctgcagaaagaagtacaattcctaacagaataatgctagcccagcactttgaggggacaacaaaggactaaggaaaaaaaattggacttaataatagactccaggtggacttagcctaagtgccactcccttaaagcctccctgccctcaaaggtggctaaaagggttttaacactgacttttagttgccaatcactcctgccaatgcaggatgcaggaccagaccaataacccgggaaaggtctattctgtcaccaagggacaatcaaagcctaactacaagatgattcatcatagatactttcggaaaaacatcttcatcaagagagggaaaggtgaaagctgtcagaatcaagagtcatgtttccaaaagccctgacaaatggagccagggaagtccatgaagagagggattttacgcactacctcaaagacccagaagaaaccacgccagcttgcacaaacactattcgcaaccttacacagaaaatacttttgggacatctgcctagaagccgattgtccaaacccgaactggcagcatccttgttattaatccttgtagccaagaataattatttcaagacaattatataatctttatctgtcctttaaaaacctgtcttcctttaccttcctgaatacacacagtttactatggcatgcatattgccttcacaatgccctattcccaaataaacatcattttcttttagaaagcctctgttatttaggttgacagttattacacctgaaaactaaattctagctgatcaataaaattctttggttctactgtatacttttatttggggatatctgcttccaaacacactaaagtacagtatactcaattttaaatatagacagtatatttaaaaaaaacataaaaagtatgtcgaacatttttaatttcaaacaccaaacttaaatagactaataacacagatcttctgtggtccacaaatcatggcaaaaaactttgttttcatatgcccattatggcttgctgactggcttactgcattttagattttccttatgattttagtagctttctctaatggaatgtgctgtgagtgaagcttcaaacattttccattgaatatacacagacatacaaataaagactggaaaaaatatacaccagtcgttttctctggttgttggaatctgggtgattttttaaagtcccatccactgggctgccagtaaaagaccacaaaatatttttgtgtatttacaggaacgtgataatcaaaagttgttgtgggaccattcaagatgagcgtggggaagggaagcccatttaaacatatattcaaggaaaaatatattaagttacctgaacatttgggtagaaatactgagcactgctatggtctgtctcccaaactgtccctcaaatgtatgatgagattttatcttcattgtggtggtgttgagagctggggcctagtgggagatgtttggttcactgaggcagatgcttcatgaatggcttggtgctgctcttgcaatgagttctcactctctcaagactagattagtccccaggagtgggttgttaaaaagagacttgtttggttgttgtgaacaagtgggttgtttgcacgtctgcttcccctctgaccttctccatcaagctatgaagcagcagcaaagcccttgccaaaagccagggccatgcccttgaacttcccagcctgtagaactgtgagcatccttcataagtgaccctgcctcagctatcctgttatagtaacacaaaacagactaagacaggcacacaaaagctgaggactgctgtcgactccactttcaagggctaccaagcacagccacatcaccaaagagaacaattcctgacctccttggaagcagaaacttgactctccgggcaagataactgttgtctttttaaaatttcagtgtcaaagttaaaacatgccttgatcagtcaaccaaattactgctaaaccagtattgggaagcttcctaaagcactccaagctcctaaaaacaggcagcatgaagtaaagcagatagcatctttgcatttaagaagtcccagaaaggttttggaaatggcattaatgtaaatgttcacattaagagaaaacggtttccctgaattgagtgattctttctactttctagtgctgtacaggataggctcagcgtttggagagtgttaacttccagtcatgtgataatggccaggagcaaccacaatgattaacctttagatagaaaacacaatcctttgcttttgtcttccttatgtatattagattaggcttctactcaatgctctgtaagttaaaacatttcaaaccaaataggccactctattaagtcccagcttgagcattcttcagcttctccacattttccattgtttgctggcaaaccagtacagtaacctgttaaatacaaagcaagggtgtggtagattgactgcatttaaggctccaattcttcacccctcctatgttctctcccttggtctaataactctgtagtgcctttccacactgggtttagccatgtggcttgtttctggtgaatgctagttagcatgaagcatgcagacatgaaagggagttatgggattgggcttggctgttgttgccttctacaacctccacaaaaacatgcttgtttaatggaggataggaggcatgtggaaaaatgccaagtccttccaggtgaggccaactccctcatgaacgaggaaagactacaactgctccagagacatctagccgaaatcacttatctaattcataaactgtttattgctgcacaccactgggtttttgtggttgctacgagttacttttgcggcaataattgctccaatatgttctatgtgacatttctgagtttaacatcacatttacaaactttcttagagaaagatttgttattagcaaagaccttcagagtaacctttgcctggtattctagactgtgcagatttagccatctaatactgagtacccacttcaggctgaatgatctctcaagtgctctcatttagttctcataaccaccctaaaaactaacttcctcattttagggaactggaggaaatgaagaactttaaggtagactgatgaaaagatttatctaaagtcacataaattggcacaatcagggtccaaaccccaggcctccgattctgagtcaaactgcattttccattacatcggaaatgaccaaggattaaaattagcagaatgttattctgtccagccattaaaatccaaaaaaaaaatttgttcaaagtaggcaattgagttttcattctattatccaaggtaactgaagtatttgactgtacaggactgcttccttcaagtgttccatccttagcattcttgttaaaaatggcctttaagatattgctattcccagtcaagaaatacccagacaactaaagagactaaaatcatgtaaatcatccatttcccagttgaatcttaaaaaaaaatttatgctcaatacctctctccagccaatcactatgtaaattgtgaattaagacattattacttggtggcaataacggttagaaaaaaagcacatccctctccctctcccgtctccccccgtctcccactttctacggtctcccactttccaccgtctccctctgatgccgagccaaggctggactgtactgccgccatctcggctcactgcaacctccctgcctgattctcctgcctcagcctgccgagtgcctgggattgcagacgcgcgccgccacgcctgactggtttttgtattttttggtggagacggggtttcgccgtgttggccaggctggtctccagctcctgaccgcgcatgatctgcccgcctgggcctcccgaggtgctgggattgcagatggagtctcgctcactcagtgctcaatgttgcccaggctggagtgcagtggcacgatctcggctcgctacaacctccacctcccagccgcctgccttggcctcccaaagtgcggagattgcagcctctgcccggccgccaccccgtctgggaagtgaggagcatctctgcctggctgcccatcgtctgggatgtgaggagcccctcagcccggccgcccagtctgggaagtgaggagcgcctcttcccggccgcccatcgtctgagatgtggggagcgcctctgccccgccgccccgtctgggatgtgaggagtgtctctgcccgaccgccaccccgtctgggaggtgaggagcgtctctgcccggccgccccgtctgagaagtgaggagcccctccgcccagcaaccaccccgtccgggaagtaaggagcgtctccgcccagcagccgccccgtctgggagggaggtggggggcagcccctgctcggccagccgccccgtccgggaggtggggggcaacccccgcccggccagctgccccgttcgggaggtggggggcagcccccggccagcatccaccccgtccgggaggtgggggggcgcctctgcccagccgccccgtctgggaagtgaggagcccctctgcccggccgccaccctgtctgggaggtgtacccaacagctcattgagagcgggccatgatgacgatggcggttttgtcgaatagaaaagggggaaatgtggggaaaggaaagagagatcagattgttgctgtgtctgtgtagaaagaagtagacataggagactccattttgttctgtactaggaaaaattcttctgccttgggatgctgttaatctataaccttacccccaaccccgtgctctctgaaacatgtgctgtgtccactcagggttaaatggattaagggcggtgcaagatgtgctttgttaaacagatgcttgaaggcagcatgctcgttaagagtcatcaccactccttaatctcaagtacccagggacacaaacactgcagaaggccgcagggtcctctgcctaggaaaaccagagacccttgttcacatgtttatctgctgaccttccctccactattgtcctatgaccctgccacatccccctctccgagaaacacccaagaatgatcaataaatactaaaaaaaaaaaaaaaaaaaaaaaaaaagactttagttcaagttgagaccaaagactgtgctattatggggtggagaaaagtatcacaattttggtaatactaggcaagatgtaacctcaagtctccaggcagccccatgagcttccctgtgaatgagaacagaaaaagttcaggagccaccagaggatgttaaggaggcttcctagagaagacgtggcaatgcacctgatggagacgtttaatttcttcactacaaggaatttcaaacttatctaaaaggaaatagaatacaacaaagctcccttacccaatcccaacaaacaaccatcaatgtcctattcattcatacctccatctacttcctctgtcacatactattttgaagcaagtcttacccattgtattttacccataaatgtttcattctgtatctctaaaacattgtctctagacctcagcaaaaaaaaaaaagcacatccacttttacaatggtcacatacaaatggggaaagagtggatataaaaaatatgcacccaccttcaatcaaatgcgatcttttaaagaatataaacaagccagattcttaggtatctctcccttttgtaattttgattctgaaaaaatatttaaagtaatcaattaggtattctaaaagaaggcagttttctaggggtttatttaattataggggggttggggtagagagattaaaaacgggaagcagtgcataggcagtatgaagtagacactttggcaaataaaaactgcaccgtatgacatgtcacatagaaattgttagagactttgaatcctaaaatttagtttaccaaatgtagctttttatgttttatgttttaccaacaaataatttgtatgttaaatttaagcatctgaattccgaaatgataaagaacaggaaaataatgactaagctaacaaccaaactttcagagtataaaattttgtcagtggttttcattttagaattaaaaatttgaatttccctttgcctacaagtctaagtaacttgcagcagcaaattcccccactgacaacttcaaagcatagcaagaatccacagtggtttgcaggccactaattcttttacagatgaaagcattcaattatctctataaaattcaattccttagaatatgtgtttgtgattgacgatgtacatttttaaatgtggtgataacacgttattattcatgatttaaaagttgaaatgaagtagcttgtggttcttgggtaaaacagacactaataagttttttttcaatataaaagagcaacctagacattcctataaaacatttttattccaggtggtaagctggcttaaattttcacttttcagccaggcatgatggctcacgcctgtaattccagcactttgggaggccgaggcaggcaaatcatctgaggtcaggagttcaagaccagcctggcaaacatggtgaaaccctgtctccactaaaaatacaaaaagtagttgggcgtggtggtgtgtgcctgtaatcccagctactcaggaggctaaggcaggagaatcacttgaacccaggaggcgaggctgcagtgagccgagatcgccccactgcaccccagcctgggcaacagagcaagactctgtctccaaaaaaaaaaaaaaaaaattcgtttttctcacagcagcacatttctaaatggcaaaccatttagaagtgagtcatcatttgtattaaaatcttatttacatggtacttatgtagtttgatcaaatactgccacaatatagtttagaggcaagacctctcatgaagaaaaactttacaagatttaaaatcagagcaaatgaatttcttaagttcaagatacgtactctcaatggagaatcgctgttgggcagtggttaaggcctctgatttgctacttattagaaaaatccacatatatacaaaactctgctaaaattccaatggcttctctagatgaatcatctttggctgtgagcaaaaaagttaactaagtttcacttaatacacacacacacactagggtttatatgtagcaacttcctcatcctcattccacaggtagcccgttcttggctgggttatggcttgtaatctcagaaccactgcccccaaatgactgctcagaagcacaatctcactgcaaactatggaacccaaactatacagctatccttggcttttaactccaagctatctaggccttgtgattatatgtgggcttcatagcagaacctaccaggcttgtggttatcaattttctgctcaccatataagcagtagctcaataacaccgtccagttttcatgtatatccagacacacaggtgagagttctgttccaagatctcattttgaccttcttcaaaggtcttctccatctctccaaattgaatgtattcttcaaccctgggcttactgtattctgcccatcttcttcctggaccaaactgttcagaagttaacttctttttcctgtcatcacatctctttcctaaactactttagaacttaaataattttattttcacataacatttagaaaggtgcagaggcagccaacaaaactattgaagacagactgtaaaaactggcaaatccccatctcaaattccatttattctataaccaataaagtcatgcagtttggacgggagcacagtaatacattctgttctcatgtagcttcctaagtatgcttagtctattgttcatttatcactgaatctgttatctgctaagtctgattcaatgttcttgccttctattaatgtgattttaagaattactgcatgtctcactatggcaaaatagcatgacatttgttttacaaaatcagttaaaccaattctacaaatatttccatacctatttattgcagcaaaagataatttttatgtgtaaattagctttttgggtttttctattcctttatttgtaaacttataatttttaggttgggcttactattttgatgagaagggtgaatctgtcaaagggtaagctggataactgtatgttgcaaacatgttcctgaacattcttcacccaaacttagacaaacctggagcttaaaataattacattggatgacatcagtttgatactgatgcctgcttcctgcactaagaggctttcaatctattttgaagagggaaaaacagaatatgccaagtggggagacagcccaaacatagaccttaatacttctctcatactcttcagccatttgatgaacatgtggaattatggatgctagggccattataaaaatctcctgatacagaacagtgtcactacttcaagctaagcagtgacaggcaaagccaggctgaggtgacaatgtagaaggatctcgagtcagccctcaatgttgttgttcaatgttgggaagtcccttttagattatttatacagtggcaggtggtagcaattacagtaaattttcttgggtttcttcctaataaaaaagtgttgataaaactacaccagtcccaaggctattcaatgccacgtaaaatagtgtattttagcatttgaggtccctttttgttgcatactaaagcatgtttaaaatggtttgcagaaaacagtctgctaaccagtactgattcatccacagaactgaattcttgcaaggcacaaaggaagtgtggctgacctaaatatttctcatttttaaaattattcatactgattatatgagattatatcttatctagtatttttcaatggagccttaaaaatgttattttgttaaaagtatatttcagcaaatttcaactttgaagatgtttttgtttacagcatagatcttatgtattagagcgctaatgtagcataggcaaactctgaaataaataaaaatgtataaatagcactgtgcagtgtgtggtgtgcgcctgttgtggggttatattaagtagtataaatttatctcccggggggataggataatcttttatgtaacaccaaattaaaaaaacaaaaacatgtactcttaaaatcatatgtccatatgtgaaatacaatcactttttttggtttccatataatttagggagtgaacaccaaaatgtaatcccatataaaaaaagatcagtttaaataaaaattaaaacaattaaaaattagtcccatagtaacatggtaaacaactcaaatggctttcttttaatgctaggaaaactgtccacctttcaacggtgacagggctgttaacacaggtaagagcaaacaaggtaaaaagtgaaagcacatacagatgatgcacacaaatatatataaaaattgaccagaaatcacaggacatgtaagcaatgttttcttaagcagaactttttttgtactttaaatagactaaaatatttggtgtaggtgggagaaagacatcagtattcaacaattttaacttgaaaaccagctgtaataaagcctcagctcattgtttaataaaaataaaaaaggaaccacatcgtacttttgacaatcatagaacgaaagctcacaaagaacacatttaatatctccatcacagtgcaccaaggatgcagccactaaggacttccagagggaaacaagaacagggtctgcatccatcatattgcattacaaagttaatgccatcagagaaaaaaaatctcacctcacgtgctcaatgttctagctggtaagcaccttatgagtatgaggctacaattgagagaaactgctcagtctgcatcaggacacccaattccttcacttgccattggctgatgcatttaatcattttaacacaacattcacggaaaaatgttaacaacacattctggcttctcgagcagaacagactgggaaatgcagtagacgccagagcatcaaaggccatgtatttcctcacaagaaaagaaatctgcaacaattggtttccttttactatgaaaaatgtaaatttcagattaagtttaaccccataaggacgcatgatttgtacttacatatacacataggttcagaagaacttagctatctagttggcctcttctctgttccattataacatcagttaccttagctggatcactaagtgtgagtctcaccaccatactggtaccttcagctattacctgtgttataaatctcatgttccattcaaagtactaaatgactggatggcacatatcccaataagtatcagaaatgttgacagccatagtgcagctgagtttagaagcaactatgacaacatagggaagtaaggataaatcacaagaacacctaaggtggtcagctccttctggtgtgcctgggacttgttttgagtttagcaaaaactttacaagattaaaaatcagagcaaatgaatttcttaagttcaagatatgtactctcaatggagaatcgcttttgggcagtggttaaggcctctgatgtgctacttatcagaaaaatccacatatatacaaaactctgctaaaagttttgtatccagggaaagtcccgcatccagggaaaccctcaatcccaggcactttagggcagctggtcaccctgagaacactacccactcgttccttaatatcactagagaaaaggtaagaactttcaagggcataacctttaagggcatcagtccccaaaatatttttacatcactagctaatggctagttcctctaagcttgctaaaaggctaggaagtccagaaataccttaaacgtgttaactttaagaagagttggtagtaatcaagcaaattagtgagcagtgtataaaagctcactcttgaaatctgttttcagacaaatcttctaaaggttcttctagctttgtccagttatatggtattttactgtattctctttttgcaattaatccagttttgtatgtcttttctttcttttttaggtgaaaatattctatgccaactgttttccacagtcctgcattatatattaaaacaaaggctgccagctggagacacagccctccgattacaaaggcccagaatgttacttttaactgtgctccaccaggaggtctggccttgggaaaagatggcgaaaggaatattctcagatatgaacattttttattctgcctacaatgctgtgatctagttcaacaactgcagaactgttctcatcttaatcgctgtagtttttctttctttactcttttgtataaaaggttagtgtcacagcttcactatcactaataaaaagatacaaatatgcctttcaagtcagggttggaaaagcaaaactgaggtgtgaggttacactggtctaagaaagtaccaatttgggttctatattttgtcaaacagttgggtttttaaaaaaattcaaaactcatgcatgttacctacttgtcatgtgtgaattatttctcacaattttaattaatctgtgtgtatattagttatataaagcaatggatttccacattcttaaagcaggaacctatattcaccagaaaaggatcctcctgtttctcatcaaattttttttcagctcgaacaatccaagattgggaatagtaagagtggcaaacaaatgttttcttagggacttactgagaaaagaaaaaacttactgggagaacagagacttagtaaaatttctattgctacagacaaatgctaaaaaccagctttataataacagcattataaaggatagaacttaatatagaaccagaaatatggcaagttacctagtgattaacattgtaaaatagtcaaaaactttaaagccacagagaaaggaaaacaattatgaaatggaaaatatataatatttaagtacttttataattctaaaacttcacttttgtccttaaatcaatatattacggatttcattgttcaataaattaccatctttaattaaaaataagtaaatcaaagagcatatttggagaaactaagagctgttaactgtttggagggtaaaagaatacttttctcgaaatttttttgaagaaaaatctaaaagccctctatgttgagttaatacaccttctgacccccatcatcagtggcattattcttccaagggactcttatatctaagcaatggtgaagttctggattcattatggatctcatggcaccaaaccaactggcactgaagttaagttaatatactccagcgagatcacctgtgggtcaaggatggcccagagaatcttggaaaatccatttatattgagcaaagatctgaatcaccttcaatcaggctgtaagatactagaaaatttgaccttgtagtagtatttcccagggtaacttaagcagcaaccttgcaccagaagaagaattaaagagggagcaatctagtattatcaacaacaacaaagttaaccctaagttagtacatcccagaatctgctggatgtataataatttagtaacggggtatatggcagagctttctttgatgttaacaaattttggctgtgattcttagttaccaagttgccaaaaaatggtatattaaatgaactgccaaatggcagattaagaaaattaatgtactccaatggtctgtccatgaaaggaaaatgtacacagacaaattaagaacattttaccaggatctgagatttaaacaatggaacaattgttttaactgttagaatgaccccaactgttaagtttgtctatgagtgtatatgtatatataaattcatacacatatattatttatttccttcttaaaaagactgaggcagttctgctatatatagttagctacaatattcaagataaaacagttcctactcaaaaaattacatgaacacacgagataagttcttatcgtaaatgctatcatgaggctatctagtatagctcatatttcctggttgtaaggctcaaaacacaggaattccactccaagagataatttgcccctcaatccctacaaagtgtagtctaaacaaacaaaatggtaataaaaaattgaaaaggaagatataaaaagaactcaatagcaggattctgactacctctggagaccacacactatcattattctgactgtcttaaatacaacaatccaatatgccccaagatggaaatctggtatcgtagggaaaacattggctgcaactgtcagaaaagttcataatcttaaacataatttatgccatttgccagtcacaaagacatttactgaacagaatttttgagccatttgtaaaattaaaatgattgatcaatttgaatagcaaccttcatgatgaagaaattaggactctaggtatgaaaagcatgttccttttttgttaataagttcaaaggagagaaacattctgatatatgcagataaaaatatggctaggctgggcgcggtggctcatgcctgtaatcccagcactttgggaagccgaggtggacagatcacgaggtcaggagatcgagaccatcctggccaacacggtgaaaccccgtctctactaaaaatacaaaaaattagccgagtgtggtggtgggcgcctgtagtcccagctacttgggaggctgaggcagaagcatggcgtgaacccgggaggcggagcttgcagtgaaccaagatcgcaccactgcactccaggttgggcaacagagcgagactccctctcaaaaaaaaaaaaaaaaaacaaaaaacaaggctaacaagaaagaggataaccagcaagtaccacctggatgtgtgttgtcaggtagaaaggaagaataaaattcaggcaatgaatataatagatttagcaaagtaaagcatatgaaaggaagaaatgtttgatatgtctaagtatcaatgccttcgatcagagtaagaaaaaagtattcattgttcatgtccacagactagatatctaaagagatacttggtgggcaggggcttgggagggaaggcgcaaattggaatgttcagcttttaaagtaaagactgtacatgaagacatattttatgtacagtgaagattgtcttgtgttactttatatcccaacataaacctacgccaccctcagacgaagagggtatctaacactgaataaatgctgaacctatttagtagttaaagaaaaaagagaaggatcttaaaggtatatatgggaagcttttaagaggtagagaaaccaactgggtatatattttcttttatttgatttcaactagcaagagactaagactgatgtttgtttgtttgttttaccttcaaagtcttagtcttaaattgacaagggcacaaaaaaagtgaaattaaaataattttaacaaaagggaaagcatttgacagtgtttaaaagacagacaaatcaagcaaaactcaatgtggcttaaggtaaaaaatacaactaggtattaaacaatttgtaaaaacttacaaagaaaatttagctttcaagaaaaattaggcagatttccttctgccaaagtgacaggtcctgaggaaaaaaaacacaacctctacaagaccaagcacagctcaagggtcagggccccgtcctagtcatctttttattattcaatatccatcacagtggctgggcaaacaacaggcatcaataaatgtttactaactgaatgtgtattataaggtataatcggtataactgatatagctcaaatctaatcatgaaagcttctttaaagtaggataaaaagagcacaatcagcggtattccagaaggtaggcctaaatccagttatatttttctaatcgttgaccagtggttataaagactttctgagcttctttttaaagcaatgaaactctttccaaaagaaaccccatgcagttcttcagtacagaataaatatgccactaagtcagtgagaactccaacagcctcccctaagccagcccccaaggtgtctctgtggaacctactggaaaaaatattactcatcttagaaatgtgatagaaagcatggccattcggttctcaggtcatcattcctagaaaattaacagtattgtgaagaataaatcctaagtaatgttgctaatttaaataaagacaaaaattcaacaaagaggggattctatcacttagaaaaatgaaaaccacacctataaatggggggaggggcagaaaacaaaaaaaaaatcaggccacagtagataaaatacaaaaaacatcatctcgttaaaaagcatcaaacacattcacacaaatgtaattacaaccaggaagtaaactgctcaacaggtataactgctcaataggtgttttcaaagagttgagtcccaatttcatactgtacagaaaaatcgcatcagaactgtagagatgcgctccactactgaaacagcatagtaggcactgcttgacctaacacagtaatgcaagagtaaccaccaagatcaggaccttctaccactttcagagttgttttctgcccctacaactgttccctaacaccattacaagttctcaagtaagaaaaagaagggcagaggctccactgagtatctcctacaggcctgatagtggtattacctaggacatttactctgctcacaagatgggtagtggaagacataattactggacagcacaaagtctggaagcaagcagcagggcactaaaacagtgagagcttacacaacaaaagcttgttaaattaagtagtactgatgtggtgcaaatgaaatttttacagcaaaggttgaggaaggagatatgttagtgagaatcacatgaagcagactatcacaaaataaggccaccttcaaaatgttatgaactgtagaaccattctgatcttcaagtttggatttgtatagaggtttctgtataaagcattaatacctaatcaggagtttcctttagtgtgaacctttttgcatttgatgctattctctttgccaggaatgcttatctcccctggctcctcacttggcttgcttctttaatgtcaggtgttagctcatgcatcctttccttagaggctttccttgatgtcctacctgaagcatcccatctgttattctccagtacagtaccctgtttatctccttcatagacaagtaagataattaagggttagtgtaactgctgtctcagcaaaggcaggaactgtagttgtcttgttcacctttacccaaagactaagaaaagttcctggtacaaacaggtgaacaataaatatttgttgaatgaataaaaaattactataccaaatttacatgaacacatacatatacacacaaatataggaaaatggggagtacccaatagaaaaccaccaaatgttgaaagtattgaaaatgatacctatagagacaggtggatatgatttcaaagaacaagtaccaaagacagcttcaaaaatatgaaaatttatgaaaagacgaccaggagtggttattttccatttctactaagatgcaaacaagaagaaatgtttaaactgcaatgagtcaacatcagacataataattatttgctgcagaatgaactagcaacagagtttcggaaatctcctctcactacagagcatgaaatattgtcaatcacaaaaccaggatcagttaagaacagctcagactgcaggtaacttataagctaaaaaacttgctaaataaatggcttttcccccaatttttaaaattctgaattcataattatgtgtagaataacaatcaatttataaactgaatacaacatactttaaaaacagatggcccatatctgctgatcctacctcagcatcacttttctaggtattttgcagaaacaattacatttacaaaaggcccatttcataatgcaatctggttactaaaccaaatcaaactactcgaagagcagaaggtctgctgttgaaatattgtaaaatacctttggaaaaacggtatttatagattagcttttttaaaaagggataaatatgtggaagtaattctagcatatccctgaaaataattatactgccacctatgcattttttatgaggtggaaggataaatcaacagactgctagattatacaagccaattattcctgttgaaatttgggcataagacaaagggactttctccatatgaattcttactgtatcccagaattaactggtgccagcagtatcaatgcaactattactggtgatgatgtcatgttatgctgttttgattatgaggacaaaaatgggaatggaaaaaagaggcttggaaaggttttcagtatggtttccttataataagatttagcagttaaaaaaaaaaacaaaaaaaaacaaaaaaccacaaaaagaatgactgtttaagccccactgaacacattaaggtcaaggatttcaaaagttaatccacttttcttcccccaagagtttatttttggtaaaaggcagaaaaattagtttttctacaggaaaatctgcttctaaataatttgaaaatcttgatatatattatatattaaaaaagacacacaaaaataacagagaagtgggaataacagattaggtactgcaactttataaaggtttgcctagatcaagaagcagcgcacacacacacctcatctatgcaaactaaaaatgtatataaacagcacaatactgtgatactggatcatgatacattacctgtacacataactactactgttattaataaacctttgggacactcagttttatgcccaataagacatcattaagtctttaaaatcttctcttcctctttaatgggagagtatttctagacactaattttcccatctaatattcaaatataggaaacagattccacaaggtgctttaattgatgagacctcaagtgctgttttctctcttgaacttttggatagtaaacagtccatagggaccacacacaatgctatgacagaagagttgttacattaagtcttttcatgggacttgattggtgaagctttatgacatgcttgagcaacgcactgaaggggatcccatctgagttaatactttgtccaaccactgtagaggtccattcagatgaagttcaatccagcaaggagtacttgttaccgtctgccttcggtattctgctccccaccctttcacaaaactcattcttatggtgcacattctagttagctgatagacggcttcaaaaccctgattaacagactgagccagaagagcagcaaattcctggttgttgaagatcttcagattacagcctggtggaattttacacactgttgcagggtgccagccatatctctgattacaattggggctctgcacaaagattgcactatcacttaggcactcagcaaaaacttccccacctatgtagtataagcgcactcctcttcctatatgccttcttgtcatttctaccgtggcatttcggttaacattggagagtaaacctaagcagaacctctctgaatttgatgggtctgtaaagccatctacagtgagtgagggctgtgatgcatggaaggtttctccaaccctctgatttaattcataatatgctatcgaacaccaaaatgcaggttctgagtaagtaactggctgtaaatccaagctatgattaacaggggaaagagtagtaggagatagttctgctggagagcctgtgtccatactttgattcaactgttggtcacttgtttctccatcttcactgatatatccaggaggtggcgtttctggaatataattactctgtggctcaattcctgctgggaagttagtgttttctggaatggagtgagtatagtcatccagaggcggaagttctgttaggatctcggtgtgtcggggcactaatactggaggcaaaactggtgtctcaactctctgatagtggtaagggtttacacatacttcatcctttttaagattaaaagcatattcgcagttttcaattgccttgagttcatgatgactgtgaagatcaggccagcgccataatcggcaatatataacatgtggcaatccttttcgatgggatacctggagacgaccatcaagagacctggtttgttcagagaagctgtaaaggcctgttgtatcccactgatctatcgtatttggtgtactcagtccccaaatttcagagcaagtgcttggtatggtaacacatttagtattacagttttgagtggtgatggctttctcaagctcatctaatcgtcctgttttctttagcttcttcaccagacttttcactgctttctcacaccacttttcttcctgcccattctgctctcctccgcctgctcctccagacccaccagctgacttcttccatcccagcagtctcttcacaactggcggcgtgaatggcaagatggacgacatgttcttaccaaaggcagcaagccacgctaggaaaacagcctcttgtatcgaacctcccggcggctggcgggctgctggctggcgagctgcttctccgccgccgcggccgcgcgggtagacccgcct

SEQ ID NO: 15518 - RNA, 29912 nt, Homo sapiens
  source 1..29912: mol_type = other RNA
gctgggattacaggcatgagccactgtacccggccccacaatttttttttttttttttttttggagagatgggatcttgctatgttgatcaggctggaaacctgggtcttgaataatggatacatttggaagtgcagagcaaaggccagagagatatccaagccagagagatatccaaggcagaacaaagctcataatttaacaagaaaggtaggcatagataggcctaattatgatgaatgctctcttaccagtataaacaaattacaaagggagtgatgagaagaggcaatgaagtttggggagggaaagaaaagtctgtggtggaggtgataacctgaacttggctttgaggaataaagagttttatatcagggcatcaagagaaggatattcaaggtacttaggaccagaacaggcaaaggcactgaagcaagagagtctggggcaagaatgtctctattgggtcaagactttgacaatattaaagattccattttcttcatatatgcccccctgctgtctttccaataaaggtaagccctgaagcctgacagtcacaggaaaggagagggtgtgtactagagtaacagcacagttgctactcagctgtgaatctcagagcctgcctttattatcttgattattctttggcatctctaggaagatgataagtagtcttcaaagtcagactttactgagaatgagaagggagttctacatgctaagagctccattcacatactaaaagcaaagcttggacaactgaacatgagttttactcctaaccatggataagagaaactgagaatacgatgtgagaagagtctcttcattaggcaggagtggaatgactcccagggcagggagagattgattgagattgcaattgccctgttgggaaataaacggaaacttcaggatgggtatgcgagtcttggagcagcagggttagtcaactactttcctggcatagcctggggaagactgcaagccactcaaaaaagtcctactcatgacttagaggcttacccagtatggcacaggagcactagctcagcattggtggaaggaggtgtctagtcagtctgagaaaatgttggcttcccaaagcttgagcaagatgttcagtacatcccaaagttccaacatcatcccttcccacccactccaaagcccagcagattaacagtcccatagttgggacatggaagctattaaggtagagaccttgagaccaaaggcaatgacagagttgtggtcaggagcagggcatgacagcagtgaacaaaagccagggacccacttacattacccagtagactcagtgacatccagcaaagatggcaggatgagcaccagcagcaggaccgtcaaggacctcagcacatacattagagaaactctttcctgtgtcacctggagatgactgttctcacccactagatgccatcatgaggaagaagctaggaagaacctttgaaaagctgagcatttatccaaagagatggttttaagcctgagataggctatttgaatcgaaagagaacgttatctttgattggcaagtttaaggccatccacctcgtcccacaccttcccaaaaccagatgggatgcatgagaaattgatgtgaaatgaaggaactgtaacttcttttctgcatgatctgagttttaatgtgtgggagctgggaagagggaagaacattgatagaaaatctgaaagcccacagggaatgtggtctaaagcagaggtttaagtcctggctgataatcattttgggttttctgaaaatgcagatcccagtgctccaattccagacctgctaaagcagaatctcacaattgaggccagggaacctacattttagaagctctccttctgactccaatttggaaaccatttatttaaccactagtacaaaaactggccttgaataagacatcacttcctccaagtctgagtacagcacgcaagggcaactgcagcaaatggaggggtgatttagtaaggagggggtgaaaccgaaaatcaacaaggtttgtgtgaactggtctcgacacacttggctgtgaatagcagggatagaaagtagttatggggcttgcaaggacattgtcttaattttcctgttgtcttaacagaggatttactgagcccatgtatgctgtaggaaaaagctagtggtgccagagtttaagttttcagaggaggaataattgacctatgtatgagttctagagaagccttgcagacttacccagggctcagagcacatggcttagtcctgacataaaataccatttttcctctaccacttggctaagaagctgaggaggaactggcagtgagggaggaggttgagaatgaaagttctggagagtcacctaagagacggtaaacacatacctcatgtcttggcttctagagcccggagataagatcagcttcccttgaaaatgttagctcccatgccacatttagtcaagacaacaataacaaaaggctttcttcagggagggcagtggaagtgagtttgagataaaaaggaatttatttatttgcacctatgtattgttcagaagttttaggtcttatgaaaaaaagatttttataaattatacacaattgggtagctttaaaaaataccaaaatatacagtggtcaccctaaaactaacatttttggataatacacttataaattggaaaatgagaaaagatagtctggtataactgcctgaacaacttattaagaacattaacaagtaataacacatattttaatgtaatattgctgactaatttggcacatttaatacacgtccaatatattttctatgtactgtgaaagcttttgggaaaataaagcagcttgtgttacaaaaactgcaacctttcacaaaggttacccacaaaatacttttgcctagccactgcctgtccaacttcagagtggcaccacccttgctattgatctttgtaaccaacgacaattatttcaaaacaattatacaaccctcatttttctttaaaatctttgtcttcctttacttccctgaatacacacgtagtttaccatgacatgggtcttttttttttttttttggagacgtagttttgcactgtcgcccaggctggagtgcagtggcacatctaggctcactgcaacctccacttctcaggttcaagccaatcttctgcctcagcctcccaagtagcgggatcataggcacccaccaatacacccatctaattttttgtatttttagtagagagggggtttcactatgttggccaggctggtctcaaactcctgacctcgtgatcggcccacctcagcctcccaaagtgctgggattacaggcataagccaccgcgcacggcccatgacatgcgtatttctacagcaatgctgtattcccaaatagagttttcttttagagagcctctctctgtgttgacataaatggtgttcagcagtagaacctgaagtaggacacatttcagagagaagtggtgatctcagaatcagtatgcagtactcacaggagccctttgggctctccgcttacatagcttgtctgttctgccccagtgagtcttttctcaggcagagcctcccacttttggcagaggctttttgacttgactttggatttgtcttggttctaagaccactttaataaaggactttacatccctcctgggatgacaaaagactttttgtctttcctggcaagtcctttttgatataaagacaagtgtccctctggtttgagtactctggatttaaaaacaatttttttttagagacagtgtctcactatactgctgaggctggtcttgaactcatgggctcaagcgatcctcctgccttggcctcccaaagtgctgggattacaggcatgggccactgcgcctggctgagtactctggattctgaggcatgccttttctggtaaatttactttgggttcttctgtgtttatattattttttaatctgcatgactgggttaacacttttgggaacactgattttggtttcgtttcgatatggttacatgcatctgtaaatgatttggctcttttcccctgtttctgaacatctcccaagagcaaaaataaacattctaaattttgggcacaggatggctcttttaaagccactagggcaatcgccaccagttaaaacactggtccaaacacctgacttatctgtcaggatttacagaattttctttgctcttaagagattgagaagaaacaaaatggaaattctcaaacattaaggcatgcctgcttttctgggacttcaggtcagctatgtggcttttcctcatgcatgtttttggatcaatgaccatcatagagattgtctatgctttgtctaaactccccaagcttttttattcttagtaccaagagactgcagctatagagttgatatgtagagtcttctaagctctctaattttttttctgcctactttaaatctgctgtttctgccagtgttgagatgaaactcactccttacggcattccagccaagaacaaaaagaaaaaaaaaggtcttaaagggccttaaattaatggctttataaattataatagttccctggcaaccaacacctagaattaagaagtatcccttttaatgtaaatttaggtttgcctaataactgcttagggtgatggaacagttaattaaaggattaatagcctaaaagaactagataaatacgtataaaaattaggctctcaaacaggtcaaaatcttgagctcagggcaataatataaggtatctctggtatagcataaaaattgcttgcctgctatgcaaaggctaaaagaacaaaacaaaaacccctcatccacaactgctaaaatgcttccctgcctgcactgactagtcaaaaaaaccagaatggcaaacaaaagatttgttactaaaaattcaaggccacctggagattgttttttcttatacaattcagccagtcctagctaaaaatgtaagcatttaaatattaacattaaactcatttgaaactgaaaaaagggaaaaaaggggttggggaggtggggtaagaggttttttaaaaatccaaactgctatttaccaaaacttttggttcacagctttcataagattacctattctgcatgtttacccagctgagcaggtcccactttctcagaaatataatttgaatccaataactgtcttttataaaccagcaagcctgtattactatcgtatgactaaaattctaaaatgaaagctatgtttgtgtatgtgtatgtttaggtgtgtttacacatatgtatatatatgttgtatgttgtgtctacgtggtaaaatctggcagttggccacaaatcccttaaggaattctattcatcaaataaatgagtgctaatacaaaatatatagtaattaacacaagtgccttttagttaatataacttaaacatctgataagctggttttaaaataattggtaaatcaaaaataagtgtctttaaaatttttgcctgaatttactactcagttttatatttgtctctgttagactttttaaggtcataaaactataaactcaacttaaaaacagaatgatctttgtataactgtaagttgaactaattttgtattattgacttcagctgtgtcctctgagttactggcaaaatacctacatatttcatttttatggttcttaattgaacacatgatactcacaggtaataaaaatggttaacaggaaaataacttgaaatgactagctatgtctaatatctcagtttttataagtaatctaggaataattgttaaaaatgaattgggggccaggtgcagtggctcacgcctgtaatcctagcactttgggaggccaaggcgggcagatcacgaggtcaggagatcgagatcacggtgaaacctcgtctctactaaaaatacaaaaaattggctgggcgcggtggcgggcgcctgtagtcccagctactcgggaggctgaggcaggagaatggcatgaacccagaaggcggagcttgcagtgagccgagatcacgccactgcactccagcctgggtgacagagcgagactccgtctcaaaaaaaaaaaaaaaaaaaagaattggatggattataaacgggataagcaagggtgagacatggtggtatgcaggtatgcatctatagttccagctactcaggaaacggaggcaggaggattgtgtgagttggagtttgaggctgcagtgtgctacaattgtgcctgtgaacagccactgaactccagcctgggtaacacagcaagacattgtctctaaaaaataaaccaaaagaatgtttttaaaaataggatgttaatgaacttttcatgtaatttgaaatcttataaattaatcttcagtaaatgtctggatcatttccaaaaaaaaacaataaactgctgaaaatattagtttgttcttggcttcctaaattatagaaagactaaatatatttgggcctattaatatacaaagttataaggaaacatgtttctaaaaattataatatggttctcatttataaaatgctgatataacacttcaaaattttgcttcctaggttttcactaaaaattaaggttaataagttaaaatttgaaaatacacaattccatatacaaagtgtacccaaaaaaagatgttttgatgagaaaagttataaggcataaaaattgctttttattgggaaaaaagttgtttaaattcagagtttattagaggttgtttcaaatatggaaacaagacagaaaggaaccactaagtaggaggaggagagaaatatgaaggaagttaatgggtgtgagaatgtacctttggtaaggaaggttacaaaattaacagaataattctgtatgagtcttgcatagtaactttttatcctaaagcaggatgaccagttgtttaaggggaagtataaaacaaagcagaaagtttaagcatgtcactgaaggtctgtgcagatcatgaaatgttcatgaaggatacatttatgaaaggagttgtgtgtaatgaagttggcaataggtcagaatgaaatcataagacattgagcttacatatatacttgtacatatgtatatgtacaataatacagtatattctatacatatgctatatatttgtatatacacgatagtgtaaatgctatacatgcactatacacacacacacacacacacacacacacacacacacacacacacaaaatttggtccccaatgttagaacaaggttctttttaaggatctggtcttaataaaattgaaagaggttttaatttttaattctaaaatcagccatcttctaaaccacagtttaaatttctgccatatttccttctgagatccgtttaatttcccctagattcaggttagaaaggctgtcttttttcatttaagatggtcatttcatttcttgaggtagagttttcttcttgaagatcctgatttatatctcacaagttcaacctttgctgtatcttgctgcaccttatttgtaggtcacacatcattgcctttagctctttctccccttaagaaggtacatctttttgtttggcaggggtgataactcttaactttttcattagctcctgtaacttttttcctctggttctaactcttgctgttataacttgatactgaaatgttctgtagaaggcctagaaaagcaatgttttcctccagtataacttgattctgaattcttggctcttctcatgtttgaattgttccacgcaagcaggaaatttctcgtaatttttccaagagccatgtattctgttcaacatactagctttcttatttacattcctctataaggcgtacactcataaccttggaaatactcttcctgtgtctgattaaattcaagtaccttttcatcagattcaactttcagtatatccaaataggcttcccataagtaaaggcagtcacactgcaagagatttttctttaccattttggcaactggcctaagaaaaattttatgttctatcaagataaattcttgtgtttaagttttttttttgcttgggaaaaatgaagctttgaaaagatggtttttaaatgtatgtaactttctgcattgcttcttaagtcttttgattatcattcttgttaaatattttatagtgacctgtgatcctgtttcgaacttttgacatctttgacaggcttctctaggctcaagttctaaattaagtgtttttgacttaaaattacctttgagttttccacttgggcctctggaaagcctcagagcatgtgtatgccatctggtagagatgttagctaattaggcttctttgatgtattaaattgtatgaaaagcattgtctaatgatgtaatactagacacagttacatttatgagtatgttattgatatgagtgttccaaaattgtacgatgccgttagaaatatgtcatcagtcataattctgattatgctgtttgccacaaaaataaccaaaactctttgtctatttctggttatggtaaactctcatcagatttttaatcatggttattctaagtttttgtaattcccagttattgctttttctctaaaagcatttgcaatcagattcatggaaaagatgctaacacacttttaaatacaggttactaatcactttaataccaatggactaaatattttttcagaacttcaagaaactgatgagtccatgtaactactaattaagatcaaccacaacaaaaaaagttacatgagactaagtaactgaagatgtgtctgtgacttttatttgaagcattattgtttttttacttaaatgttttgttttccatatttaaagaaattctctcatgctatctatagtttacagcaatttggaatacttttgtgaacaaaggtagaaatatttgcttttcctttcttcttgatccctccaatttggaaactattttgagtattcatttgtttttgtttttgagacggagtctcgctctgttgccccagctggaatgcagtggcacgatcttgtttcagtgcaacttctgcctccagggttcaagcaattctgtctcagcctcccaagtagctgggactacaggcatgcaccaccacacccagctaatttttgtattttttagtagagacggtggccggggggaggtttcactatgttggccaggctggtttcaaactcctgacctcaggtgttccacctgtcttggcctcccaaagagctgggattacaggcatgagccactgtgcccagcctatttgtgagtactcttaaggcaatatgatttgcctaagttcaataaaaatcggctctcgttataacaggatacaattggaaacactggttgtattaccaaggctttgattaaaatgtcatatttgagaatgtgtagaatgcctggcttcaatggttctcagcattacactgaattaaaaattatcatttcctggcaggcccaggaaccttaaaactataggtaaaatctaaagtctaccttgacttagcttcttagcctcaaggaggtttttaaatctgagattactgtgaccatactactattcttgcagacaaaatctgataaagtttacaaatctgttttattctgaacatctttggtaaaaatcagggtaactttaagtttctgaagaaagctatatgtacctgttattagatcacagctctgtaccgttttgaaactcctgttatccacctgcagactggatttgctcctgaatcctcctaatttccttcaatatttggctatgactctctaagaaaaaaaactactcccatgctctgaggcctataagctaagatgtgattaatttttaaaggagcaagtctcatgctgatgtatgggtcacacaaaagttcaccataccaaccaatgccatagctagagacattcaaactgcaaaccaggacaaaaagttgatgatttcaggctgtagacatttttcctaagacatcagagcaagaattgtattacaatttgatttattcaattggttgcctgtaagcctaggttcagggctcaaaaccattatgcaaactgggattgtcacattactattaattttgtgtatttcctttttaaactttgtatctgttatttgccaaattttctgcagaaagaagtacaattcctaacagaataatgctagcccagcactttgaggggacaacaaaggactaaggaaaaaaaattggacttaataatagactccaggtggacttagcctaagtgccactcccttaaagcctccctgccctcaaaggtggctaaaagggttttaacactgacttttagttgccaatcactcctgccaatgcaggatgcaggaccagaccaataacccgggaaaggtctattctgtcaccaagggacaatcaaagcctaactacaagatgattcatcatagatactttcggaaaaacatcttcatcaagagagggaaaggtgaaagctgtcagaatcaagagtcatgtttccaaaagccctgacaaatggagccagggaagtccatgaagagagggattttacgcactacctcaaagacccagaagaaaccacgccagcttgcacaaacactattcgcaaccttacacagaaaatacttttgggacatctgcctagaagccgattgtccaaacccgaactggcagcatccttgttattaatccttgtagccaagaataattatttcaagacaattatataatctttatctgtcctttaaaaacctgtcttcctttaccttcctgaatacacacagtttactatggcatgcatattgccttcacaatgccctattcccaaataaacatcattttcttttagaaagcctctgttatttaggttgacagttattacacctgaaaactaaattctagctgatcaataaaattctttggttctactgtatacttttatttggggatatctgcttccaaacacactaaagtacagtatactcaattttaaatatagacagtatatttaaaaaaaacataaaaagtatgtcgaacatttttaatttcaaacaccaaacttaaatagactaataacacagatcttctgtggtccacaaatcatggcaaaaaactttgttttcatatgcccattatggcttgctgactggcttactgcattttagattttccttatgattttagtagctttctctaatggaatgtgctgtgagtgaagcttcaaacattttccattgaatatacacagacatacaaataaagactggaaaaaatatacaccagtcgttttctctggttgttggaatctgggtgattttttaaagtcccatccactgggctgccagtaaaagaccacaaaatatttttgtgtatttacaggaacgtgataatcaaaagttgttgtgggaccattcaagatgagcgtggggaagggaagcccatttaaacatatattcaaggaaaaatatattaagttacctgaacatttgggtagaaatactgagcactgctatggtctgtctcccaaactgtccctcaaatgtatgatgagattttatcttcattgtggtggtgttgagagctggggcctagtgggagatgtttggttcactgaggcagatgcttcatgaatggcttggtgctgctcttgcaatgagttctcactctctcaagactagattagtccccaggagtgggttgttaaaaagagacttgtttggttgttgtgaacaagtgggttgtttgcacgtctgcttcccctctgaccttctccatcaagctatgaagcagcagcaaagcccttgccaaaagccagggccatgcccttgaacttcccagcctgtagaactgtgagcatccttcataagtgaccctgcctcagctatcctgttatagtaacacaaaacagactaagacaggcacacaaaagctgaggactgctgtcgactccactttcaagggctaccaagcacagccacatcaccaaagagaacaattcctgacctccttggaagcagaaacttgactctccgggcaagataactgttgtctttttaaaatttcagtgtcaaagttaaaacatgccttgatcagtcaaccaaattactgctaaaccagtattgggaagcttcctaaagcactccaagctcctaaaaacaggcagcatgaagtaaagcagatagcatctttgcatttaagaagtcccagaaaggttttggaaatggcattaatgtaaatgttcacattaagagaaaacggtttccctgaattgagtgattctttctactttctagtgctgtacaggataggctcagcgtttggagagtgttaacttccagtcatgtgataatggccaggagcaaccacaatgattaacctttagatagaaaacacaatcctttgcttttgtcttccttatgtatattagattaggcttctactcaatgctctgtaagttaaaacatttcaaaccaaataggccactctattaagtcccagcttgagcattcttcagcttctccacattttccattgtttgctggcaaaccagtacagtaacctgttaaatacaaagcaagggtgtggtagattgactgcatttaaggctccaattcttcacccctcctatgttctctcccttggtctaataactctgtagtgcctttccacactgggtttagccatgtggcttgtttctggtgaatgctagttagcatgaagcatgcagacatgaaagggagttatgggattgggcttggctgttgttgccttctacaacctccacaaaaacatgcttgtttaatggaggataggaggcatgtggaaaaatgccaagtccttccaggtgaggccaactccctcatgaacgaggaaagactacaactgctccagagacatctagccgaaatcacttatctaattcataaactgtttattgctgcacaccactgggtttttgtggttgctacgagttacttttgcggcaataattgctccaatatgttctatgtgacatttctgagtttaacatcacatttacaaactttcttagagaaagatttgttattagcaaagaccttcagagtaacctttgcctggtattctagactgtgcagatttagccatctaatactgagtacccacttcaggctgaatgatctctcaagtgctctcatttagttctcataaccaccctaaaaactaacttcctcattttagggaactggaggaaatgaagaactttaaggtagactgatgaaaagatttatctaaagtcacataaattggcacaatcagggtccaaaccccaggcctccgattctgagtcaaactgcattttccattacatcggaaatgaccaaggattaaaattagcagaatgttattctgtccagccattaaaatccaaaaaaaaaatttgttcaaagtaggcaattgagttttcattctattatccaaggtaactgaagtatttgactgtacaggactgcttccttcaagtgttccatccttagcattcttgttaaaaatggcctttaagatattgctattcccagtcaagaaatacccagacaactaaagagactaaaatcatgtaaatcatccatttcccagttgaatcttaaaaaaaaatttatgctcaatacctctctccagccaatcactatgtaaattgtgaattaagacattattacttggtggcaataacggttagaaaaaaagcacatccctctccctctcccgtctccccccgtctcccactttctacggtctcccactttccaccgtctccctctgatgccgagccaaggctggactgtactgccgccatctcggctcactgcaacctccctgcctgattctcctgcctcagcctgccgagtgcctgggattgcagacgcgcgccgccacgcctgactggtttttgtattttttggtggagacggggtttcgccgtgttggccaggctggtctccagctcctgaccgcgcatgatctgcccgcctgggcctcccgaggtgctgggattgcagatggagtctcgctcactcagtgctcaatgttgcccaggctggagtgcagtggcacgatctcggctcgctacaacctccacctcccagccgcctgccttggcctcccaaagtgcggagattgcagcctctgcccggccgccaccccgtctgggaagtgaggagcatctctgcctggctgcccatcgtctgggatgtgaggagcccctcagcccggccgcccagtctgggaagtgaggagcgcctcttcccggccgcccatcgtctgagatgtggggagcgcctctgccccgccgccccgtctgggatgtgaggagtgtctctgcccgaccgccaccccgtctgggaggtgaggagcgtctctgcccggccgccccgtctgagaagtgaggagcccctccgcccagcaaccaccccgtccgggaagtaaggagcgtctccgcccagcagccgccccgtctgggagggaggtggggggcagcccctgctcggccagccgccccgtccgggaggtggggggcaacccccgcccggccagctgccccgttcgggaggtggggggcagcccccggccagcatccaccccgtccgggaggtgggggggcgcctctgcccagccgccccgtctgggaagtgaggagcccctctgcccggccgccaccctgtctgggaggtgtacccaacagctcattgagagcgggccatgatgacgatggcggttttgtcgaatagaaaagggggaaatgtggggaaaggaaagagagatcagattgttgctgtgtctgtgtagaaagaagtagacataggagactccattttgttctgtactaggaaaaattcttctgccttgggatgctgttaatctataaccttacccccaaccccgtgctctctgaaacatgtgctgtgtccactcagggttaaatggattaagggcggtgcaagatgtgctttgttaaacagatgcttgaaggcagcatgctcgttaagagtcatcaccactccttaatctcaagtacccagggacacaaacactgcagaaggccgcagggtcctctgcctaggaaaaccagagacccttgttcacatgtttatctgctgaccttccctccactattgtcctatgaccctgccacatccccctctccgagaaacacccaagaatgatcaataaatactaaaaaaaaaaaaaaaaaaaaaaaaaaagactttagttcaagttgagaccaaagactgtgctattatggggtggagaaaagtatcacaattttggtaatactaggcaagatgtaacctcaagtctccaggcagccccatgagcttccctgtgaatgagaacagaaaaagttcaggagccaccagaggatgttaaggaggcttcctagagaagacgtggcaatgcacctgatggagacgtttaatttcttcactacaaggaatttcaaacttatctaaaaggaaatagaatacaacaaagctcccttacccaatcccaacaaacaaccatcaatgtcctattcattcatacctccatctacttcctctgtcacatactattttgaagcaagtcttacccattgtattttacccataaatgtttcattctgtatctctaaaacattgtctctagacctcagcaaaaaaaaaaaagcacatccacttttacaatggtcacatacaaatggggaaagagtggatataaaaaatatgcacccaccttcaatcaaatgcgatcttttaaagaatataaacaagccagattcttaggtatctctcccttttgtaattttgattctgaaaaaatatttaaagtaatcaattaggtattctaaaagaaggcagttttctaggggtttatttaattataggggggttggggtagagagattaaaaacgggaagcagtgcataggcagtatgaagtagacactttggcaaataaaaactgcaccgtatgacatgtcacatagaaattgttagagactttgaatcctaaaatttagtttaccaaatgtagctttttatgttttatgttttaccaacaaataatttgtatgttaaatttaagcatctgaattccgaaatgataaagaacaggaaaataatgactaagctaacaaccaaactttcagagtataaaattttgtcagtggttttcattttagaattaaaaatttgaatttccctttgcctacaagtctaagtaacttgcagcagcaaattcccccactgacaacttcaaagcatagcaagaatccacagtggtttgcaggccactaattcttttacagatgaaagcattcaattatctctataaaattcaattccttagaatatgtgtttgtgattgacgatgtacatttttaaatgtggtgataacacgttattattcatgatttaaaagttgaaatgaagtagcttgtggttcttgggtaaaacagacactaataagttttttttcaatataaaagagcaacctagacattcctataaaacatttttattccaggtggtaagctggcttaaattttcacttttcagccaggcatgatggctcacgcctgtaattccagcactttgggaggccgaggcaggcaaatcatctgaggtcaggagttcaagaccagcctggcaaacatggtgaaaccctgtctccactaaaaatacaaaaagtagttgggcgtggtggtgtgtgcctgtaatcccagctactcaggaggctaaggcaggagaatcacttgaacccaggaggcgaggctgcagtgagccgagatcgccccactgcaccccagcctgggcaacagagcaagactctgtctccaaaaaaaaaaaaaaaaaattcgtttttctcacagcagcacatttctaaatggcaaaccatttagaagtgagtcatcatttgtattaaaatcttatttacatggtacttatgtagtttgatcaaatactgccacaatatagtttagaggcaagacctctcatgaagaaaaactttacaagatttaaaatcagagcaaatgaatttcttaagttcaagatacgtactctcaatggagaatcgctgttgggcagtggttaaggcctctgatttgctacttattagaaaaatccacatatatacaaaactctgctaaaattccaatggcttctctagatgaatcatctttggctgtgagcaaaaaagttaactaagtttcacttaatacacacacacacactagggtttatatgtagcaacttcctcatcctcattccacaggtagcccgttcttggctgggttatggcttgtaatctcagaaccactgcccccaaatgactgctcagaagcacaatctcactgcaaactatggaacccaaactatacagctatccttggcttttaactccaagctatctaggccttgtgattatatgtgggcttcatagcagaacctaccaggcttgtggttatcaattttctgctcaccatataagcagtagctcaataacaccgtccagttttcatgtatatccagacacacaggtgagagttctgttccaagatctcattttgaccttcttcaaaggtcttctccatctctccaaattgaatgtattcttcaaccctgggcttactgtattctgcccatcttcttcctggaccaaactgttcagaagttaacttctttttcctgtcatcacatctctttcctaaactactttagaacttaaataattttattttcacataacatttagaaaggtgcagaggcagccaacaaaactattgaagacagactgtaaaaactggcaaatccccatctcaaattccatttattctataaccaataaagtcatgcagtttggacgggagcacagtaatacattctgttctcatgtagcttcctaagtatgcttagtctattgttcatttatcactgaatctgttatctgctaagtctgattcaatgttcttgccttctattaatgtgattttaagaattactgcatgtctcactatggcaaaatagcatgacatttgttttacaaaatcagttaaaccaattctacaaatatttccatacctatttattgcagcaaaagataatttttatgtgtaaattagctttttgggtttttctattcctttatttgtaaacttataatttttaggttgggcttactattttgatgagaagggtgaatctgtcaaagggtaagctggataactgtatgttgcaaacatgttcctgaacattcttcacccaaacttagacaaacctggagcttaaaataattacattggatgacatcagtttgatactgatgcctgcttcctgcactaagaggctttcaatctattttgaagagggaaaaacagaatatgccaagtggggagacagcccaaacatagaccttaatacttctctcatactcttcagccatttgatgaacatgtggaattatggatgctagggccattataaaaatctcctgatacagaacagtgtcactacttcaagctaagcagtgacaggcaaagccaggctgaggtgacaatgtagaaggatctcgagtcagccctcaatgttgttgttcaatgttgggaagtcccttttagattatttatacagtggcaggtggtagcaattacagtaaattttcttgggtttcttcctaataaaaaagtgttgataaaactacaccagtcccaaggctattcaatgccacgtaaaatagtgtattttagcatttgaggtccctttttgttgcatactaaagcatgtttaaaatggtttgcagaaaacagtctgctaaccagtactgattcatccacagaactgaattcttgcaaggcacaaaggaagtgtggctgacctaaatatttctcatttttaaaattattcatactgattatatgagattatatcttatctagtatttttcaatggagccttaaaaatgttattttgttaaaagtatatttcagcaaatttcaactttgaagatgtttttgtttacagcatagatcttatgtattagagcgctaatgtagcataggcaaactctgaaataaataaaaatgtataaatagcactgtgcagtgtgtggtgtgcgcctgttgtggggttatattaagtagtataaatttatctcccggggggataggataatcttttatgtaacaccaaattaaaaaaacaaaaacatgtactcttaaaatcatatgtccatatgtgaaatacaatcactttttttggtttccatataatttagggagtgaacaccaaaatgtaatcccatataaaaaaagatcagtttaaataaaaattaaaacaattaaaaattagtcccatagtaacatggtaaacaactcaaatggctttcttttaatgctaggaaaactgtccacctttcaacggtgacagggctgttaacacaggtaagagcaaacaaggtaaaaagtgaaagcacatacagatgatgcacacaaatatatataaaaattgaccagaaatcacaggacatgtaagcaatgttttcttaagcagaactttttttgtactttaaatagactaaaatatttggtgtaggtgggagaaagacatcagtattcaacaattttaacttgaaaaccagctgtaataaagcctcagctcattgtttaataaaaataaaaaaggaaccacatcgtacttttgacaatcatagaacgaaagctcacaaagaacacatttaatatctccatcacagtgcaccaaggatgcagccactaaggacttccagagggaaacaagaacagggtctgcatccatcatattgcattacaaagttaatgccatcagagaaaaaaaatctcacctcacgtgctcaatgttctagctggtaagcaccttatgagtatgaggctacaattgagagaaactgctcagtctgcatcaggacacccaattccttcacttgccattggctgatgcatttaatcattttaacacaacattcacggaaaaatgttaacaacacattctggcttctcgagcagaacagactgggaaatgcagtagacgccagagcatcaaaggccatgtatttcctcacaagaaaagaaatctgcaacaattggtttccttttactatgaaaaatgtaaatttcagattaagtttaaccccataaggacgcatgatttgtacttacatatacacataggttcagaagaacttagctatctagttggcctcttctctgttccattataacatcagttaccttagctggatcactaagtgtgagtctcaccaccatactggtaccttcagctattacctgtgttataaatctcatgttccattcaaagtactaaatgactggatggcacatatcccaataagtatcagaaatgttgacagccatagtgcagctgagtttagaagcaactatgacaacatagggaagtaaggataaatcacaagaacacctaaggtggtcagctccttctggtgtgcctgggacttgttttgagtttagcaaaaactttacaagattaaaaatcagagcaaatgaatttcttaagttcaagatatgtactctcaatggagaatcgcttttgggcagtggttaaggcctctgatgtgctacttatcagaaaaatccacatatatacaaaactctgctaaaagttttgtatccagggaaagtcccgcatccagggaaaccctcaatcccaggcactttagggcagctggtcaccctgagaacactacccactcgttccttaatatcactagagaaaaggtaagaactttcaagggcataacctttaagggcatcagtccccaaaatatttttacatcactagctaatggctagttcctctaagcttgctaaaaggctaggaagtccagaaataccttaaacgtgttaactttaagaagagttggtagtaatcaagcaaattagtgagcagtgtataaaagctcactcttgaaatctgttttcagacaaatcttctaaaggttcttctagctttgtccagttatatggtattttactgtattctctttttgcaattaatccagttttgtatgtcttttctttcttttttaggtgaaaatattctatgccaactgttttccacagtcctgcattatatattaaaacaaaggctgccagctggagacacagccctccgattacaaaggcccagaatgttacttttaactgtgctccaccaggaggtctggccttgggaaaagatggcgaaaggaatattctcagatatgaacattttttattctgcctacaatgctgtgatctagttcaacaactgcagaactgttctcatcttaatcgctgtagtttttctttctttactcttttgtataaaaggttagtgtcacagcttcactatcactaataaaaagatacaaatatgcctttcaagtcagggttggaaaagcaaaactgaggtgtgaggttacactggtctaagaaagtaccaatttgggttctatattttgtcaaacagttgggtttttaaaaaaattcaaaactcatgcatgttacctacttgtcatgtgtgaattatttctcacaattttaattaatctgtgtgtatattagttatataaagcaatggatttccacattcttaaagcaggaacctatattcaccagaaaaggatcctcctgtttctcatcaaattttttttcagctcgaacaatccaagattgggaatagtaagagtggcaaacaaatgttttcttagggacttactgagaaaagaaaaaacttactgggagaacagagacttagtaaaatttctattgctacagacaaatgctaaaaaccagctttataataacagcattataaaggatagaacttaatatagaaccagaaatatggcaagttacctagtgattaacattgtaaaatagtcaaaaactttaaagccacagagaaaggaaaacaattatgaaatggaaaatatataatatttaagtacttttataattctaaaacttcacttttgtccttaaatcaatatattacggatttcattgttcaataaattaccatctttaattaaaaataagtaaatcaaagagcatatttggagaaactaagagctgttaactgtttggagggtaaaagaatacttttctcgaaatttttttgaagaaaaatctaaaagccctctatgttgagttaatacaccttctgacccccatcatcagtggcattattcttccaagggactcttatatctaagcaatggtgaagttctggattcattatggatctcatggcaccaaaccaactggcactgaagttaagttaatatactccagcgagatcacctgtgggtcaaggatggcccagagaatcttggaaaatccatttatattgagcaaagatctgaatcaccttcaatcaggctgtaagatactagaaaatttgaccttgtagtagtatttcccagggtaacttaagcagcaaccttgcaccagaagaagaattaaagagggagcaatctagtattatcaacaacaacaaagttaaccctaagttagtacatcccagaatctgctggatgtataataatttagtaacggggtatatggcagagctttctttgatgttaacaaattttggctgtgattcttagttaccaagttgccaaaaaatggtatattaaatgaactgccaaatggcagattaagaaaattaatgtactccaatggtctgtccatgaaaggaaaatgtacacagacaaattaagaacattttaccaggatctgagatttaaacaatggaacaattgttttaactgttagaatgaccccaactgttaagtttgtctatgagtgtatatgtatatataaattcatacacatatattatttatttccttcttaaaaagactgaggcagttctgctatatatagttagctacaatattcaagataaaacagttcctactcaaaaaattacatgaacacacgagataagttcttatcgtaaatgctatcatgaggctatctagtatagctcatatttcctggttgtaaggctcaaaacacaggaattccactccaagagataatttgcccctcaatccctacaaagtgtagtctaaacaaacaaaatggtaataaaaaattgaaaaggaagatataaaaagaactcaatagcaggattctgactacctctggagaccacacactatcattattctgactgtcttaaatacaacaatccaatatgccccaagatggaaatctggtatcgtagggaaaacattggctgcaactgtcagaaaagttcataatcttaaacataatttatgccatttgccagtcacaaagacatttactgaacagaatttttgagccatttgtaaaattaaaatgattgatcaatttgaatagcaaccttcatgatgaagaaattaggactctaggtatgaaaagcatgttccttttttgttaataagttcaaaggagagaaacattctgatatatgcagataaaaatatggctaggctgggcgcggtggctcatgcctgtaatcccagcactttgggaagccgaggtggacagatcacgaggtcaggagatcgagaccatcctggccaacacggtgaaaccccgtctctactaaaaatacaaaaaattagccgagtgtggtggtgggcgcctgtagtcccagctacttgggaggctgaggcagaagcatggcgtgaacccgggaggcggagcttgcagtgaaccaagatcgcaccactgcactccaggttgggcaacagagcgagactccctctcaaaaaaaaaaaaaaaaaacaaaaaacaaggctaacaagaaagaggataaccagcaagtaccacctggatgtgtgttgtcaggtagaaaggaagaataaaattcaggcaatgaatataatagatttagcaaagtaaagcatatgaaaggaagaaatgtttgatatgtctaagtatcaatgccttcgatcagagtaagaaaaaagtattcattgttcatgtccacagactagatatctaaagagatacttggtgggcaggggcttgggagggaaggcgcaaattggaatgttcagcttttaaagtaaagactgtacatgaagacatattttatgtacagtgaagattgtcttgtgttactttatatcccaacataaacctacgccaccctcagacgaagagggtatctaacactgaataaatgctgaacctatttagtagttaaagaaaaaagagaaggatcttaaaggtatatatgggaagcttttaagaggtagagaaaccaactgggtatatattttcttttatttgatttcaactagcaagagactaagactgatgtttgtttgtttgttttaccttcaaagtcttagtcttaaattgacaagggcacaaaaaaagtgaaattaaaataattttaacaaaagggaaagcatttgacagtgtttaaaagacagacaaatcaagcaaaactcaatgtggcttaaggtaaaaaatacaactaggtattaaacaatttgtaaaaacttacaaagaaaatttagctttcaagaaaaattaggcagatttccttctgccaaagtgacaggtcctgaggaaaaaaaacacaacctctacaagaccaagcacagctcaagggtcagggccccgtcctagtcatctttttattattcaatatccatcacagtggctgggcaaacaacaggcatcaataaatgtttactaactgaatgtgtattataaggtataatcggtataactgatatagctcaaatctaatcatgaaagcttctttaaagtaggataaaaagagcacaatcagcggtattccagaaggtaggcctaaatccagttatatttttctaatcgttgaccagtggttataaagactttctgagcttctttttaaagcaatgaaactctttccaaaagaaaccccatgcagttcttcagtacagaataaatatgccactaagtcagtgagaactccaacagcctcccctaagccagcccccaaggtgtctctgtggaacctactggaaaaaatattactcatcttagaaatgtgatagaaagcatggccattcggttctcaggtcatcattcctagaaaattaacagtattgtgaagaataaatcctaagtaatgttgctaatttaaataaagacaaaaattcaacaaagaggggattctatcacttagaaaaatgaaaaccacacctataaatggggggaggggcagaaaacaaaaaaaaaatcaggccacagtagataaaatacaaaaaacatcatctcgttaaaaagcatcaaacacattcacacaaatgtaattacaaccaggaagtaaactgctcaacaggtataactgctcaataggtgttttcaaagagttgagtcccaatttcatactgtacagaaaaatcgcatcagaactgtagagatgcgctccactactgaaacagcatagtaggcactgcttgacctaacacagtaatgcaagagtaaccaccaagatcaggaccttctaccactttcagagttgttttctgcccctacaactgttccctaacaccattacaagttctcaagtaagaaaaagaagggcagaggctccactgagtatctcctacaggcctgatagtggtattacctaggacatttactctgctcacaagatgggtagtggaagacataattactggacagcacaaagtctggaagcaagcagcagggcactaaaacagtgagagcttacacaacaaaagcttgttaaattaagtagtactgatgtggtgcaaatgaaatttttacagcaaaggttgaggaaggagatatgttagtgagaatcacatgaagcagactatcacaaaataaggccaccttcaaaatgttatgaactgtagaaccattctgatcttcaagtttggatttgtatagaggtttctgtataaagcattaatacctaatcaggagtttcctttagtgtgaacctttttgcatttgatgctattctctttgccaggaatgcttatctcccctggctcctcacttggcttgcttctttaatgtcaggtgttagctcatgcatcctttccttagaggctttccttgatgtcctacctgaagcatcccatctgttattctccagtacagtaccctgtttatctccttcatagacaagtaagataattaagggttagtgtaactgctgtctcagcaaaggcaggaactgtagttgtcttgttcacctttacccaaagactaagaaaagttcctggtacaaacaggtgaacaataaatatttgttgaatgaataaaaaattactataccaaatttacatgaacacatacatatacacacaaatataggaaaatggggagtacccaatagaaaaccaccaaatgttgaaagtattgaaaatgatacctatagagacaggtggatatgatttcaaagaacaagtaccaaagacagcttcaaaaatatgaaaatttatgaaaagacgaccaggagtggttattttccatttctactaagatgcaaacaagaagaaatgtttaaactgcaatgagtcaacatcagacataataattatttgctgcagaatgaactagcaacagagtttcggaaatctcctctcactacagagcatgaaatattgtcaatcacaaaaccaggatcagttaagaacagctcagactgcaggtaacttataagctaaaaaacttgctaaataaatggcttttcccccaatttttaaaattctgaattcataattatgtgtagaataacaatcaatttataaactgaatacaacatactttaaaaacagatggcccatatctgctgatcctacctcagcatcacttttctaggtattttgcagaaacaattacatttacaaaaggcccatttcataatgcaatctggttactaaaccaaatcaaactactcgaagagcagaaggtctgctgttgaaatattgtaaaatacctttggaaaaacggtatttatagattagcttttttaaaaagggataaatatgtggaagtaattctagcatatccctgaaaataattatactgccacctatgcattttttatgaggtggaaggataaatcaacagactgctagattatacaagccaattattcctgttgaaatttgggcataagacaaagggactttctccatatgaattcttactgtatcccagaattaactggtgccagcagtatcaatgcaactattactggtgatgatgtcatgttatgctgttttgattatgaggacaaaaatgggaatggaaaaaagaggcttggaaaggttttcagtatggtttccttataataagatttagcagttaaaaaaaaaaacaaaaaaaaacaaaaaaccacaaaaagaatgactgtttaagccccactgaacacattaaggtcaaggatttcaaaagttaatccacttttcttcccccaagagtttatttttggtaaaaggcagaaaaattagtttttctacaggaaaatctgcttctaaataatttgaaaatcttgatatatattatatattaaaaaagacacacaaaaataacagagaagtgggaataacagattaggtactgcaactttataaaggtttgcctagatcaagaagcagcgcacacacacacctcatctatgcaaactaaaaatgtatataaacagcacaatactgtgatactggatcatgatacattacctgtacacataactactactgttattaataaacctttgggacactcagttttatgcccaataagacatcattaagtctttaaaatcttctcttcctctttaatgggagagtatttctagacactaattttcccatctaatattcaaatataggaaacagattccacaaggtgctttaattgatgagacctcaagtgctgttttctctcttgaacttttggatagtaaacagtccatagggaccacacacaatgctatgacagaagagttgttacattaagtcttttcatgggacttgattggtgaagctttatgacatgcttgagcaacgcactgaaggggatcccatctgagttaatactttgtccaaccactgtagaggtccattcagatgaagttcaatccagcaaggagtacttgttaccgtctgccttcggtattctgctccccaccctttcacaaaactcattcttatggtgcacattctagttagctgatagacggcttcaaaaccctgattaacagactgagccagaagagcagcaaattcctggttgttgaagatcttcagattacagcctggtggaattttacacactgttgcagggtgccagccatatctctgattacaattggggctctgcacaaagattgcactatcacttaggcactcagcaaaaacttccccacctatgtagtataagcgcactcctcttcctatatgccttcttgtcatttctaccgtggcatttcggttaacattggagagtaaacctaagcagaacctctctgaatttgatgggtctgtaaagccatctacagtgagtgagggctgtgatgcatggaaggtttctccaaccctctgatttaattcataatatgctatcgaacaccaaaatgcaggttctgagtaagtaactggctgtaaatccaagctatgattaacaggggaaagagtagtaggagatagttctgctggagagcctgtgtccatactttgattcaactgttggtcacttgtttctccatcttcactgatatatccaggaggtggcgtttctggaatataattactctgtggctcaattcctgctgggaagttagtgttttctggaatggagtgagtatagtcatccagaggcggaagttctgttaggatctcggtgtgtcggggcactaatactggaggcaaaactggtgtctcaactctctgatagtggtaagggtttacacatacttcatcctttttaagattaaaagcatattcgcagttttcaattgccttgagttcatgatgactgtgaagatcaggccagcgccataatcggcaatatataacatgtggcaatccttttcgatgggatacctggagacgaccatcaagagacctggtttgttcagagaagctgtaaaggcctgttgtatcccactgatctatcgtatttggtgtactcagtccccaaatttcagagcaagtgcttggtatggtaacacatttagtattacagttttgagtggtgatggctttctcaagctcatctaatcgtcctgttttctttagcttcttcaccagacttttcactgctttctcacaccacttttcttcctgcccattctgctctcctccgcctgctcctccagacccaccagctgacttcttccatcccagcagtctcttcacaactggcggcgtgaatggcaagatggacgacatgttcttaccaaaggcagcaagccacgctaggaaaacagcctcttgtatcgaacctgcaaggtggcgccaggtcccgccccgtcagatccggggggtccgggaccttttgttccttcctcttccgatgggatggagggggctgggaggggaagaggggaatgggcgattggaggcggaactgaaaacactcccggccgccgtcttcccgccccgcccccaggcccgggcccggccggcggcccgggcgcgcgggagggtaggggaagagaggggaggggaggggaggagagggaaggggaggggagggagcctggccgccgcccgcggggaaggagggggtgaggacgcgcgc

SEQ ID NO: 15519 - RNA, 29596 nt, Homo sapiens
  source 1..29596: mol_type = other RNA
gctgggattacaggcatgagccactgtacccggccccacaatttttttttttttttttttttggagagatgggatcttgctatgttgatcaggctggaaacctgggtcttgaataatggatacatttggaagtgcagagcaaaggccagagagatatccaagccagagagatatccaaggcagaacaaagctcataatttaacaagaaaggtaggcatagataggcctaattatgatgaatgctctcttaccagtataaacaaattacaaagggagtgatgagaagaggcaatgaagtttggggagggaaagaaaagtctgtggtggaggtgataacctgaacttggctttgaggaataaagagttttatatcagggcatcaagagaaggatattcaaggtacttaggaccagaacaggcaaaggcactgaagcaagagagtctggggcaagaatgtctctattgggtcaagactttgacaatattaaagattccattttcttcatatatgcccccctgctgtctttccaataaaggtaagccctgaagcctgacagtcacaggaaaggagagggtgtgtactagagtaacagcacagttgctactcagctgtgaatctcagagcctgcctttattatcttgattattctttggcatctctaggaagatgataagtagtcttcaaagtcagactttactgagaatgagaagggagttctacatgctaagagctccattcacatactaaaagcaaagcttggacaactgaacatgagttttactcctaaccatggataagagaaactgagaatacgatgtgagaagagtctcttcattaggcaggagtggaatgactcccagggcagggagagattgattgagattgcaattgccctgttgggaaataaacggaaacttcaggatgggtatgcgagtcttggagcagcagggttagtcaactactttcctggcatagcctggggaagactgcaagccactcaaaaaagtcctactcatgacttagaggcttacccagtatggcacaggagcactagctcagcattggtggaaggaggtgtctagtcagtctgagaaaatgttggcttcccaaagcttgagcaagatgttcagtacatcccaaagttccaacatcatcccttcccacccactccaaagcccagcagattaacagtcccatagttgggacatggaagctattaaggtagagaccttgagaccaaaggcaatgacagagttgtggtcaggagcagggcatgacagcagtgaacaaaagccagggacccacttacattacccagtagactcagtgacatccagcaaagatggcaggatgagcaccagcagcaggaccgtcaaggacctcagcacatacattagagaaactctttcctgtgtcacctggagatgactgttctcacccactagatgccatcatgaggaagaagctaggaagaacctttgaaaagctgagcatttatccaaagagatggttttaagcctgagataggctatttgaatcgaaagagaacgttatctttgattggcaagtttaaggccatccacctcgtcccacaccttcccaaaaccagatgggatgcatgagaaattgatgtgaaatgaaggaactgtaacttcttttctgcatgatctgagttttaatgtgtgggagctgggaagagggaagaacattgatagaaaatctgaaagcccacagggaatgtggtctaaagcagaggtttaagtcctggctgataatcattttgggttttctgaaaatgcagatcccagtgctccaattccagacctgctaaagcagaatctcacaattgaggccagggaacctacattttagaagctctccttctgactccaatttggaaaccatttatttaaccactagtacaaaaactggccttgaataagacatcacttcctccaagtctgagtacagcacgcaagggcaactgcagcaaatggaggggtgatttagtaaggagggggtgaaaccgaaaatcaacaaggtttgtgtgaactggtctcgacacacttggctgtgaatagcagggatagaaagtagttatggggcttgcaaggacattgtcttaattttcctgttgtcttaacagaggatttactgagcccatgtatgctgtaggaaaaagctagtggtgccagagtttaagttttcagaggaggaataattgacctatgtatgagttctagagaagccttgcagacttacccagggctcagagcacatggcttagtcctgacataaaataccatttttcctctaccacttggctaagaagctgaggaggaactggcagtgagggaggaggttgagaatgaaagttctggagagtcacctaagagacggtaaacacatacctcatgtcttggcttctagagcccggagataagatcagcttcccttgaaaatgttagctcccatgccacatttagtcaagacaacaataacaaaaggctttcttcagggagggcagtggaagtgagtttgagataaaaaggaatttatttatttgcacctatgtattgttcagaagttttaggtcttatgaaaaaaagatttttataaattatacacaattgggtagctttaaaaaataccaaaatatacagtggtcaccctaaaactaacatttttggataatacacttataaattggaaaatgagaaaagatagtctggtataactgcctgaacaacttattaagaacattaacaagtaataacacatattttaatgtaatattgctgactaatttggcacatttaatacacgtccaatatattttctatgtactgtgaaagcttttgggaaaataaagcagcttgtgttacaaaaactgcaacctttcacaaaggttacccacaaaatacttttgcctagccactgcctgtccaacttcagagtggcaccacccttgctattgatctttgtaaccaacgacaattatttcaaaacaattatacaaccctcatttttctttaaaatctttgtcttcctttacttccctgaatacacacgtagtttaccatgacatgggtcttttttttttttttttggagacgtagttttgcactgtcgcccaggctggagtgcagtggcacatctaggctcactgcaacctccacttctcaggttcaagccaatcttctgcctcagcctcccaagtagcgggatcataggcacccaccaatacacccatctaattttttgtatttttagtagagagggggtttcactatgttggccaggctggtctcaaactcctgacctcgtgatcggcccacctcagcctcccaaagtgctgggattacaggcataagccaccgcgcacggcccatgacatgcgtatttctacagcaatgctgtattcccaaatagagttttcttttagagagcctctctctgtgttgacataaatggtgttcagcagtagaacctgaagtaggacacatttcagagagaagtggtgatctcagaatcagtatgcagtactcacaggagccctttgggctctccgcttacatagcttgtctgttctgccccagtgagtcttttctcaggcagagcctcccacttttggcagaggctttttgacttgactttggatttgtcttggttctaagaccactttaataaaggactttacatccctcctgggatgacaaaagactttttgtctttcctggcaagtcctttttgatataaagacaagtgtccctctggtttgagtactctggatttaaaaacaatttttttttagagacagtgtctcactatactgctgaggctggtcttgaactcatgggctcaagcgatcctcctgccttggcctcccaaagtgctgggattacaggcatgggccactgcgcctggctgagtactctggattctgaggcatgccttttctggtaaatttactttgggttcttctgtgtttatattattttttaatctgcatgactgggttaacacttttgggaacactgattttggtttcgtttcgatatggttacatgcatctgtaaatgatttggctcttttcccctgtttctgaacatctcccaagagcaaaaataaacattctaaattttgggcacaggatggctcttttaaagccactagggcaatcgccaccagttaaaacactggtccaaacacctgacttatctgtcaggatttacagaattttctttgctcttaagagattgagaagaaacaaaatggaaattctcaaacattaaggcatgcctgcttttctgggacttcaggtcagctatgtggcttttcctcatgcatgtttttggatcaatgaccatcatagagattgtctatgctttgtctaaactccccaagcttttttattcttagtaccaagagactgcagctatagagttgatatgtagagtcttctaagctctctaattttttttctgcctactttaaatctgctgtttctgccagtgttgagatgaaactcactccttacggcattccagccaagaacaaaaagaaaaaaaaaggtcttaaagggccttaaattaatggctttataaattataatagttccctggcaaccaacacctagaattaagaagtatcccttttaatgtaaatttaggtttgcctaataactgcttagggtgatggaacagttaattaaaggattaatagcctaaaagaactagataaatacgtataaaaattaggctctcaaacaggtcaaaatcttgagctcagggcaataatataaggtatctctggtatagcataaaaattgcttgcctgctatgcaaaggctaaaagaacaaaacaaaaacccctcatccacaactgctaaaatgcttccctgcctgcactgactagtcaaaaaaaccagaatggcaaacaaaagatttgttactaaaaattcaaggccacctggagattgttttttcttatacaattcagccagtcctagctaaaaatgtaagcatttaaatattaacattaaactcatttgaaactgaaaaaagggaaaaaaggggttggggaggtggggtaagaggttttttaaaaatccaaactgctatttaccaaaacttttggttcacagctttcataagattacctattctgcatgtttacccagctgagcaggtcccactttctcagaaatataatttgaatccaataactgtcttttataaaccagcaagcctgtattactatcgtatgactaaaattctaaaatgaaagctatgtttgtgtatgtgtatgtttaggtgtgtttacacatatgtatatatatgttgtatgttgtgtctacgtggtaaaatctggcagttggccacaaatcccttaaggaattctattcatcaaataaatgagtgctaatacaaaatatatagtaattaacacaagtgccttttagttaatataacttaaacatctgataagctggttttaaaataattggtaaatcaaaaataagtgtctttaaaatttttgcctgaatttactactcagttttatatttgtctctgttagactttttaaggtcataaaactataaactcaacttaaaaacagaatgatctttgtataactgtaagttgaactaattttgtattattgacttcagctgtgtcctctgagttactggcaaaatacctacatatttcatttttatggttcttaattgaacacatgatactcacaggtaataaaaatggttaacaggaaaataacttgaaatgactagctatgtctaatatctcagtttttataagtaatctaggaataattgttaaaaatgaattgggggccaggtgcagtggctcacgcctgtaatcctagcactttgggaggccaaggcgggcagatcacgaggtcaggagatcgagatcacggtgaaacctcgtctctactaaaaatacaaaaaattggctgggcgcggtggcgggcgcctgtagtcccagctactcgggaggctgaggcaggagaatggcatgaacccagaaggcggagcttgcagtgagccgagatcacgccactgcactccagcctgggtgacagagcgagactccgtctcaaaaaaaaaaaaaaaaaaaagaattggatggattataaacgggataagcaagggtgagacatggtggtatgcaggtatgcatctatagttccagctactcaggaaacggaggcaggaggattgtgtgagttggagtttgaggctgcagtgtgctacaattgtgcctgtgaacagccactgaactccagcctgggtaacacagcaagacattgtctctaaaaaataaaccaaaagaatgtttttaaaaataggatgttaatgaacttttcatgtaatttgaaatcttataaattaatcttcagtaaatgtctggatcatttccaaaaaaaaacaataaactgctgaaaatattagtttgttcttggcttcctaaattatagaaagactaaatatatttgggcctattaatatacaaagttataaggaaacatgtttctaaaaattataatatggttctcatttataaaatgctgatataacacttcaaaattttgcttcctaggttttcactaaaaattaaggttaataagttaaaatttgaaaatacacaattccatatacaaagtgtacccaaaaaaagatgttttgatgagaaaagttataaggcataaaaattgctttttattgggaaaaaagttgtttaaattcagagtttattagaggttgtttcaaatatggaaacaagacagaaaggaaccactaagtaggaggaggagagaaatatgaaggaagttaatgggtgtgagaatgtacctttggtaaggaaggttacaaaattaacagaataattctgtatgagtcttgcatagtaactttttatcctaaagcaggatgaccagttgtttaaggggaagtataaaacaaagcagaaagtttaagcatgtcactgaaggtctgtgcagatcatgaaatgttcatgaaggatacatttatgaaaggagttgtgtgtaatgaagttggcaataggtcagaatgaaatcataagacattgagcttacatatatacttgtacatatgtatatgtacaataatacagtatattctatacatatgctatatatttgtatatacacgatagtgtaaatgctatacatgcactatacacacacacacacacacacacacacacacacacacacacacacaaaatttggtccccaatgttagaacaaggttctttttaaggatctggtcttaataaaattgaaagaggttttaatttttaattctaaaatcagccatcttctaaaccacagtttaaatttctgccatatttccttctgagatccgtttaatttcccctagattcaggttagaaaggctgtcttttttcatttaagatggtcatttcatttcttgaggtagagttttcttcttgaagatcctgatttatatctcacaagttcaacctttgctgtatcttgctgcaccttatttgtaggtcacacatcattgcctttagctctttctccccttaagaaggtacatctttttgtttggcaggggtgataactcttaactttttcattagctcctgtaacttttttcctctggttctaactcttgctgttataacttgatactgaaatgttctgtagaaggcctagaaaagcaatgttttcctccagtataacttgattctgaattcttggctcttctcatgtttgaattgttccacgcaagcaggaaatttctcgtaatttttccaagagccatgtattctgttcaacatactagctttcttatttacattcctctataaggcgtacactcataaccttggaaatactcttcctgtgtctgattaaattcaagtaccttttcatcagattcaactttcagtatatccaaataggcttcccataagtaaaggcagtcacactgcaagagatttttctttaccattttggcaactggcctaagaaaaattttatgttctatcaagataaattcttgtgtttaagttttttttttgcttgggaaaaatgaagctttgaaaagatggtttttaaatgtatgtaactttctgcattgcttcttaagtcttttgattatcattcttgttaaatattttatagtgacctgtgatcctgtttcgaacttttgacatctttgacaggcttctctaggctcaagttctaaattaagtgtttttgacttaaaattacctttgagttttccacttgggcctctggaaagcctcagagcatgtgtatgccatctggtagagatgttagctaattaggcttctttgatgtattaaattgtatgaaaagcattgtctaatgatgtaatactagacacagttacatttatgagtatgttattgatatgagtgttccaaaattgtacgatgccgttagaaatatgtcatcagtcataattctgattatgctgtttgccacaaaaataaccaaaactctttgtctatttctggttatggtaaactctcatcagatttttaatcatggttattctaagtttttgtaattcccagttattgctttttctctaaaagcatttgcaatcagattcatggaaaagatgctaacacacttttaaatacaggttactaatcactttaataccaatggactaaatattttttcagaacttcaagaaactgatgagtccatgtaactactaattaagatcaaccacaacaaaaaaagttacatgagactaagtaactgaagatgtgtctgtgacttttatttgaagcattattgtttttttacttaaatgttttgttttccatatttaaagaaattctctcatgctatctatagtttacagcaatttggaatacttttgtgaacaaaggtagaaatatttgcttttcctttcttcttgatccctccaatttggaaactattttgagtattcatttgtttttgtttttgagacggagtctcgctctgttgccccagctggaatgcagtggcacgatcttgtttcagtgcaacttctgcctccagggttcaagcaattctgtctcagcctcccaagtagctgggactacaggcatgcaccaccacacccagctaatttttgtattttttagtagagacggtggccggggggaggtttcactatgttggccaggctggtttcaaactcctgacctcaggtgttccacctgtcttggcctcccaaagagctgggattacaggcatgagccactgtgcccagcctatttgtgagtactcttaaggcaatatgatttgcctaagttcaataaaaatcggctctcgttataacaggatacaattggaaacactggttgtattaccaaggctttgattaaaatgtcatatttgagaatgtgtagaatgcctggcttcaatggttctcagcattacactgaattaaaaattatcatttcctggcaggcccaggaaccttaaaactataggtaaaatctaaagtctaccttgacttagcttcttagcctcaaggaggtttttaaatctgagattactgtgaccatactactattcttgcagacaaaatctgataaagtttacaaatctgttttattctgaacatctttggtaaaaatcagggtaactttaagtttctgaagaaagctatatgtacctgttattagatcacagctctgtaccgttttgaaactcctgttatccacctgcagactggatttgctcctgaatcctcctaatttccttcaatatttggctatgactctctaagaaaaaaaactactcccatgctctgaggcctataagctaagatgtgattaatttttaaaggagcaagtctcatgctgatgtatgggtcacacaaaagttcaccataccaaccaatgccatagctagagacattcaaactgcaaaccaggacaaaaagttgatgatttcaggctgtagacatttttcctaagacatcagagcaagaattgtattacaatttgatttattcaattggttgcctgtaagcctaggttcagggctcaaaaccattatgcaaactgggattgtcacattactattaattttgtgtatttcctttttaaactttgtatctgttatttgccaaattttctgcagaaagaagtacaattcctaacagaataatgctagcccagcactttgaggggacaacaaaggactaaggaaaaaaaattggacttaataatagactccaggtggacttagcctaagtgccactcccttaaagcctccctgccctcaaaggtggctaaaagggttttaacactgacttttagttgccaatcactcctgccaatgcaggatgcaggaccagaccaataacccgggaaaggtctattctgtcaccaagggacaatcaaagcctaactacaagatgattcatcatagatactttcggaaaaacatcttcatcaagagagggaaaggtgaaagctgtcagaatcaagagtcatgtttccaaaagccctgacaaatggagccagggaagtccatgaagagagggattttacgcactacctcaaagacccagaagaaaccacgccagcttgcacaaacactattcgcaaccttacacagaaaatacttttgggacatctgcctagaagccgattgtccaaacccgaactggcagcatccttgttattaatccttgtagccaagaataattatttcaagacaattatataatctttatctgtcctttaaaaacctgtcttcctttaccttcctgaatacacacagtttactatggcatgcatattgccttcacaatgccctattcccaaataaacatcattttcttttagaaagcctctgttatttaggttgacagttattacacctgaaaactaaattctagctgatcaataaaattctttggttctactgtatacttttatttggggatatctgcttccaaacacactaaagtacagtatactcaattttaaatatagacagtatatttaaaaaaaacataaaaagtatgtcgaacatttttaatttcaaacaccaaacttaaatagactaataacacagatcttctgtggtccacaaatcatggcaaaaaactttgttttcatatgcccattatggcttgctgactggcttactgcattttagattttccttatgattttagtagctttctctaatggaatgtgctgtgagtgaagcttcaaacattttccattgaatatacacagacatacaaataaagactggaaaaaatatacaccagtcgttttctctggttgttggaatctgggtgattttttaaagtcccatccactgggctgccagtaaaagaccacaaaatatttttgtgtatttacaggaacgtgataatcaaaagttgttgtgggaccattcaagatgagcgtggggaagggaagcccatttaaacatatattcaaggaaaaatatattaagttacctgaacatttgggtagaaatactgagcactgctatggtctgtctcccaaactgtccctcaaatgtatgatgagattttatcttcattgtggtggtgttgagagctggggcctagtgggagatgtttggttcactgaggcagatgcttcatgaatggcttggtgctgctcttgcaatgagttctcactctctcaagactagattagtccccaggagtgggttgttaaaaagagacttgtttggttgttgtgaacaagtgggttgtttgcacgtctgcttcccctctgaccttctccatcaagctatgaagcagcagcaaagcccttgccaaaagccagggccatgcccttgaacttcccagcctgtagaactgtgagcatccttcataagtgaccctgcctcagctatcctgttatagtaacacaaaacagactaagacaggcacacaaaagctgaggactgctgtcgactccactttcaagggctaccaagcacagccacatcaccaaagagaacaattcctgacctccttggaagcagaaacttgactctccgggcaagataactgttgtctttttaaaatttcagtgtcaaagttaaaacatgccttgatcagtcaaccaaattactgctaaaccagtattgggaagcttcctaaagcactccaagctcctaaaaacaggcagcatgaagtaaagcagatagcatctttgcatttaagaagtcccagaaaggttttggaaatggcattaatgtaaatgttcacattaagagaaaacggtttccctgaattgagtgattctttctactttctagtgctgtacaggataggctcagcgtttggagagtgttaacttccagtcatgtgataatggccaggagcaaccacaatgattaacctttagatagaaaacacaatcctttgcttttgtcttccttatgtatattagattaggcttctactcaatgctctgtaagttaaaacatttcaaaccaaataggccactctattaagtcccagcttgagcattcttcagcttctccacattttccattgtttgctggcaaaccagtacagtaacctgttaaatacaaagcaagggtgtggtagattgactgcatttaaggctccaattcttcacccctcctatgttctctcccttggtctaataactctgtagtgcctttccacactgggtttagccatgtggcttgtttctggtgaatgctagttagcatgaagcatgcagacatgaaagggagttatgggattgggcttggctgttgttgccttctacaacctccacaaaaacatgcttgtttaatggaggataggaggcatgtggaaaaatgccaagtccttccaggtgaggccaactccctcatgaacgaggaaagactacaactgctccagagacatctagccgaaatcacttatctaattcataaactgtttattgctgcacaccactgggtttttgtggttgctacgagttacttttgcggcaataattgctccaatatgttctatgtgacatttctgagtttaacatcacatttacaaactttcttagagaaagatttgttattagcaaagaccttcagagtaacctttgcctggtattctagactgtgcagatttagccatctaatactgagtacccacttcaggctgaatgatctctcaagtgctctcatttagttctcataaccaccctaaaaactaacttcctcattttagggaactggaggaaatgaagaactttaaggtagactgatgaaaagatttatctaaagtcacataaattggcacaatcagggtccaaaccccaggcctccgattctgagtcaaactgcattttccattacatcggaaatgaccaaggattaaaattagcagaatgttattctgtccagccattaaaatccaaaaaaaaaatttgttcaaagtaggcaattgagttttcattctattatccaaggtaactgaagtatttgactgtacaggactgcttccttcaagtgttccatccttagcattcttgttaaaaatggcctttaagatattgctattcccagtcaagaaatacccagacaactaaagagactaaaatcatgtaaatcatccatttcccagttgaatcttaaaaaaaaatttatgctcaatacctctctccagccaatcactatgtaaattgtgaattaagacattattacttggtggcaataacggttagaaaaaaagcacatccctctccctctcccgtctccccccgtctcccactttctacggtctcccactttccaccgtctccctctgatgccgagccaaggctggactgtactgccgccatctcggctcactgcaacctccctgcctgattctcctgcctcagcctgccgagtgcctgggattgcagacgcgcgccgccacgcctgactggtttttgtattttttggtggagacggggtttcgccgtgttggccaggctggtctccagctcctgaccgcgcatgatctgcccgcctgggcctcccgaggtgctgggattgcagatggagtctcgctcactcagtgctcaatgttgcccaggctggagtgcagtggcacgatctcggctcgctacaacctccacctcccagccgcctgccttggcctcccaaagtgcggagattgcagcctctgcccggccgccaccccgtctgggaagtgaggagcatctctgcctggctgcccatcgtctgggatgtgaggagcccctcagcccggccgcccagtctgggaagtgaggagcgcctcttcccggccgcccatcgtctgagatgtggggagcgcctctgccccgccgccccgtctgggatgtgaggagtgtctctgcccgaccgccaccccgtctgggaggtgaggagcgtctctgcccggccgccccgtctgagaagtgaggagcccctccgcccagcaaccaccccgtccgggaagtaaggagcgtctccgcccagcagccgccccgtctgggagggaggtggggggcagcccctgctcggccagccgccccgtccgggaggtggggggcaacccccgcccggccagctgccccgttcgggaggtggggggcagcccccggccagcatccaccccgtccgggaggtgggggggcgcctctgcccagccgccccgtctgggaagtgaggagcccctctgcccggccgccaccctgtctgggaggtgtacccaacagctcattgagagcgggccatgatgacgatggcggttttgtcgaatagaaaagggggaaatgtggggaaaggaaagagagatcagattgttgctgtgtctgtgtagaaagaagtagacataggagactccattttgttctgtactaggaaaaattcttctgccttgggatgctgttaatctataaccttacccccaaccccgtgctctctgaaacatgtgctgtgtccactcagggttaaatggattaagggcggtgcaagatgtgctttgttaaacagatgcttgaaggcagcatgctcgttaagagtcatcaccactccttaatctcaagtacccagggacacaaacactgcagaaggccgcagggtcctctgcctaggaaaaccagagacccttgttcacatgtttatctgctgaccttccctccactattgtcctatgaccctgccacatccccctctccgagaaacacccaagaatgatcaataaatactaaaaaaaaaaaaaaaaaaaaaaaaaaagactttagttcaagttgagaccaaagactgtgctattatggggtggagaaaagtatcacaattttggtaatactaggcaagatgtaacctcaagtctccaggcagccccatgagcttccctgtgaatgagaacagaaaaagttcaggagccaccagaggatgttaaggaggcttcctagagaagacgtggcaatgcacctgatggagacgtttaatttcttcactacaaggaatttcaaacttatctaaaaggaaatagaatacaacaaagctcccttacccaatcccaacaaacaaccatcaatgtcctattcattcatacctccatctacttcctctgtcacatactattttgaagcaagtcttacccattgtattttacccataaatgtttcattctgtatctctaaaacattgtctctagacctcagcaaaaaaaaaaaagcacatccacttttacaatggtcacatacaaatggggaaagagtggatataaaaaatatgcacccaccttcaatcaaatgcgatcttttaaagaatataaacaagccagattcttaggtatctctcccttttgtaattttgattctgaaaaaatatttaaagtaatcaattaggtattctaaaagaaggcagttttctaggggtttatttaattataggggggttggggtagagagattaaaaacgggaagcagtgcataggcagtatgaagtagacactttggcaaataaaaactgcaccgtatgacatgtcacatagaaattgttagagactttgaatcctaaaatttagtttaccaaatgtagctttttatgttttatgttttaccaacaaataatttgtatgttaaatttaagcatctgaattccgaaatgataaagaacaggaaaataatgactaagctaacaaccaaactttcagagtataaaattttgtcagtggttttcattttagaattaaaaatttgaatttccctttgcctacaagtctaagtaacttgcagcagcaaattcccccactgacaacttcaaagcatagcaagaatccacagtggtttgcaggccactaattcttttacagatgaaagcattcaattatctctataaaattcaattccttagaatatgtgtttgtgattgacgatgtacatttttaaatgtggtgataacacgttattattcatgatttaaaagttgaaatgaagtagcttgtggttcttgggtaaaacagacactaataagttttttttcaatataaaagagcaacctagacattcctataaaacatttttattccaggtggtaagctggcttaaattttcacttttcagccaggcatgatggctcacgcctgtaattccagcactttgggaggccgaggcaggcaaatcatctgaggtcaggagttcaagaccagcctggcaaacatggtgaaaccctgtctccactaaaaatacaaaaagtagttgggcgtggtggtgtgtgcctgtaatcccagctactcaggaggctaaggcaggagaatcacttgaacccaggaggcgaggctgcagtgagccgagatcgccccactgcaccccagcctgggcaacagagcaagactctgtctccaaaaaaaaaaaaaaaaaattcgtttttctcacagcagcacatttctaaatggcaaaccatttagaagtgagtcatcatttgtattaaaatcttatttacatggtacttatgtagtttgatcaaatactgccacaatatagtttagaggcaagacctctcatgaagaaaaactttacaagatttaaaatcagagcaaatgaatttcttaagttcaagatacgtactctcaatggagaatcgctgttgggcagtggttaaggcctctgatttgctacttattagaaaaatccacatatatacaaaactctgctaaaattccaatggcttctctagatgaatcatctttggctgtgagcaaaaaagttaactaagtttcacttaatacacacacacacactagggtttatatgtagcaacttcctcatcctcattccacaggtagcccgttcttggctgggttatggcttgtaatctcagaaccactgcccccaaatgactgctcagaagcacaatctcactgcaaactatggaacccaaactatacagctatccttggcttttaactccaagctatctaggccttgtgattatatgtgggcttcatagcagaacctaccaggcttgtggttatcaattttctgctcaccatataagcagtagctcaataacaccgtccagttttcatgtatatccagacacacaggtgagagttctgttccaagatctcattttgaccttcttcaaaggtcttctccatctctccaaattgaatgtattcttcaaccctgggcttactgtattctgcccatcttcttcctggaccaaactgttcagaagttaacttctttttcctgtcatcacatctctttcctaaactactttagaacttaaataattttattttcacataacatttagaaaggtgcagaggcagccaacaaaactattgaagacagactgtaaaaactggcaaatccccatctcaaattccatttattctataaccaataaagtcatgcagtttggacgggagcacagtaatacattctgttctcatgtagcttcctaagtatgcttagtctattgttcatttatcactgaatctgttatctgctaagtctgattcaatgttcttgccttctattaatgtgattttaagaattactgcatgtctcactatggcaaaatagcatgacatttgttttacaaaatcagttaaaccaattctacaaatatttccatacctatttattgcagcaaaagataatttttatgtgtaaattagctttttgggtttttctattcctttatttgtaaacttataatttttaggttgggcttactattttgatgagaagggtgaatctgtcaaagggtaagctggataactgtatgttgcaaacatgttcctgaacattcttcacccaaacttagacaaacctggagcttaaaataattacattggatgacatcagtttgatactgatgcctgcttcctgcactaagaggctttcaatctattttgaagagggaaaaacagaatatgccaagtggggagacagcccaaacatagaccttaatacttctctcatactcttcagccatttgatgaacatgtggaattatggatgctagggccattataaaaatctcctgatacagaacagtgtcactacttcaagctaagcagtgacaggcaaagccaggctgaggtgacaatgtagaaggatctcgagtcagccctcaatgttgttgttcaatgttgggaagtcccttttagattatttatacagtggcaggtggtagcaattacagtaaattttcttgggtttcttcctaataaaaaagtgttgataaaactacaccagtcccaaggctattcaatgccacgtaaaatagtgtattttagcatttgaggtccctttttgttgcatactaaagcatgtttaaaatggtttgcagaaaacagtctgctaaccagtactgattcatccacagaactgaattcttgcaaggcacaaaggaagtgtggctgacctaaatatttctcatttttaaaattattcatactgattatatgagattatatcttatctagtatttttcaatggagccttaaaaatgttattttgttaaaagtatatttcagcaaatttcaactttgaagatgtttttgtttacagcatagatcttatgtattagagcgctaatgtagcataggcaaactctgaaataaataaaaatgtataaatagcactgtgcagtgtgtggtgtgcgcctgttgtggggttatattaagtagtataaatttatctcccggggggataggataatcttttatgtaacaccaaattaaaaaaacaaaaacatgtactcttaaaatcatatgtccatatgtgaaatacaatcactttttttggtttccatataatttagggagtgaacaccaaaatgtaatcccatataaaaaaagatcagtttaaataaaaattaaaacaattaaaaattagtcccatagtaacatggtaaacaactcaaatggctttcttttaatgctaggaaaactgtccacctttcaacggtgacagggctgttaacacaggtaagagcaaacaaggtaaaaagtgaaagcacatacagatgatgcacacaaatatatataaaaattgaccagaaatcacaggacatgtaagcaatgttttcttaagcagaactttttttgtactttaaatagactaaaatatttggtgtaggtgggagaaagacatcagtattcaacaattttaacttgaaaaccagctgtaataaagcctcagctcattgtttaataaaaataaaaaaggaaccacatcgtacttttgacaatcatagaacgaaagctcacaaagaacacatttaatatctccatcacagtgcaccaaggatgcagccactaaggacttccagagggaaacaagaacagggtctgcatccatcatattgcattacaaagttaatgccatcagagaaaaaaaatctcacctcacgtgctcaatgttctagctggtaagcaccttatgagtatgaggctacaattgagagaaactgctcagtctgcatcaggacacccaattccttcacttgccattggctgatgcatttaatcattttaacacaacattcacggaaaaatgttaacaacacattctggcttctcgagcagaacagactgggaaatgcagtagacgccagagcatcaaaggccatgtatttcctcacaagaaaagaaatctgcaacaattggtttccttttactatgaaaaatgtaaatttcagattaagtttaaccccataaggacgcatgatttgtacttacatatacacataggttcagaagaacttagctatctagttggcctcttctctgttccattataacatcagttaccttagctggatcactaagtgtgagtctcaccaccatactggtaccttcagctattacctgtgttataaatctcatgttccattcaaagtactaaatgactggatggcacatatcccaataagtatcagaaatgttgacagccatagtgcagctgagtttagaagcaactatgacaacatagggaagtaaggataaatcacaagaacacctaaggtggtcagctccttctggtgtgcctgggacttgttttgagtttagcaaaaactttacaagattaaaaatcagagcaaatgaatttcttaagttcaagatatgtactctcaatggagaatcgcttttgggcagtggttaaggcctctgatgtgctacttatcagaaaaatccacatatatacaaaactctgctaaaagttttgtatccagggaaagtcccgcatccagggaaaccctcaatcccaggcactttagggcagctggtcaccctgagaacactacccactcgttccttaatatcactagagaaaaggtaagaactttcaagggcataacctttaagggcatcagtccccaaaatatttttacatcactagctaatggctagttcctctaagcttgctaaaaggctaggaagtccagaaataccttaaacgtgttaactttaagaagagttggtagtaatcaagcaaattagtgagcagtgtataaaagctcactcttgaaatctgttttcagacaaatcttctaaaggttcttctagctttgtccagttatatggtattttactgtattctctttttgcaattaatccagttttgtatgtcttttctttcttttttaggtgaaaatattctatgccaactgttttccacagtcctgcattatatattaaaacaaaggctgccagctggagacacagccctccgattacaaaggcccagaatgttacttttaactgtgctccaccaggaggtctggccttgggaaaagatggcgaaaggaatattctcagatatgaacattttttattctgcctacaatgctgtgatctagttcaacaactgcagaactgttctcatcttaatcgctgtagtttttctttctttactcttttgtataaaaggttagtgtcacagcttcactatcactaataaaaagatacaaatatgcctttcaagtcagggttggaaaagcaaaactgaggtgtgaggttacactggtctaagaaagtaccaatttgggttctatattttgtcaaacagttgggtttttaaaaaaattcaaaactcatgcatgttacctacttgtcatgtgtgaattatttctcacaattttaattaatctgtgtgtatattagttatataaagcaatggatttccacattcttaaagcaggaacctatattcaccagaaaaggatcctcctgtttctcatcaaattttttttcagctcgaacaatccaagattgggaatagtaagagtggcaaacaaatgttttcttagggacttactgagaaaagaaaaaacttactgggagaacagagacttagtaaaatttctattgctacagacaaatgctaaaaaccagctttataataacagcattataaaggatagaacttaatatagaaccagaaatatggcaagttacctagtgattaacattgtaaaatagtcaaaaactttaaagccacagagaaaggaaaacaattatgaaatggaaaatatataatatttaagtacttttataattctaaaacttcacttttgtccttaaatcaatatattacggatttcattgttcaataaattaccatctttaattaaaaataagtaaatcaaagagcatatttggagaaactaagagctgttaactgtttggagggtaaaagaatacttttctcgaaatttttttgaagaaaaatctaaaagccctctatgttgagttaatacaccttctgacccccatcatcagtggcattattcttccaagggactcttatatctaagcaatggtgaagttctggattcattatggatctcatggcaccaaaccaactggcactgaagttaagttaatatactccagcgagatcacctgtgggtcaaggatggcccagagaatcttggaaaatccatttatattgagcaaagatctgaatcaccttcaatcaggctgtaagatactagaaaatttgaccttgtagtagtatttcccagggtaacttaagcagcaaccttgcaccagaagaagaattaaagagggagcaatctagtattatcaacaacaacaaagttaaccctaagttagtacatcccagaatctgctggatgtataataatttagtaacggggtatatggcagagctttctttgatgttaacaaattttggctgtgattcttagttaccaagttgccaaaaaatggtatattaaatgaactgccaaatggcagattaagaaaattaatgtactccaatggtctgtccatgaaaggaaaatgtacacagacaaattaagaacattttaccaggatctgagatttaaacaatggaacaattgttttaactgttagaatgaccccaactgttaagtttgtctatgagtgtatatgtatatataaattcatacacatatattatttatttccttcttaaaaagactgaggcagttctgctatatatagttagctacaatattcaagataaaacagttcctactcaaaaaattacatgaacacacgagataagttcttatcgtaaatgctatcatgaggctatctagtatagctcatatttcctggttgtaaggctcaaaacacaggaattccactccaagagataatttgcccctcaatccctacaaagtgtagtctaaacaaacaaaatggtaataaaaaattgaaaaggaagatataaaaagaactcaatagcaggattctgactacctctggagaccacacactatcattattctgactgtcttaaatacaacaatccaatatgccccaagatggaaatctggtatcgtagggaaaacattggctgcaactgtcagaaaagttcataatcttaaacataatttatgccatttgccagtcacaaagacatttactgaacagaatttttgagccatttgtaaaattaaaatgattgatcaatttgaatagcaaccttcatgatgaagaaattaggactctaggtatgaaaagcatgttccttttttgttaataagttcaaaggagagaaacattctgatatatgcagataaaaatatggctaggctgggcgcggtggctcatgcctgtaatcccagcactttgggaagccgaggtggacagatcacgaggtcaggagatcgagaccatcctggccaacacggtgaaaccccgtctctactaaaaatacaaaaaattagccgagtgtggtggtgggcgcctgtagtcccagctacttgggaggctgaggcagaagcatggcgtgaacccgggaggcggagcttgcagtgaaccaagatcgcaccactgcactccaggttgggcaacagagcgagactccctctcaaaaaaaaaaaaaaaaaacaaaaaacaaggctaacaagaaagaggataaccagcaagtaccacctggatgtgtgttgtcaggtagaaaggaagaataaaattcaggcaatgaatataatagatttagcaaagtaaagcatatgaaaggaagaaatgtttgatatgtctaagtatcaatgccttcgatcagagtaagaaaaaagtattcattgttcatgtccacagactagatatctaaagagatacttggtgggcaggggcttgggagggaaggcgcaaattggaatgttcagcttttaaagtaaagactgtacatgaagacatattttatgtacagtgaagattgtcttgtgttactttatatcccaacataaacctacgccaccctcagacgaagagggtatctaacactgaataaatgctgaacctatttagtagttaaagaaaaaagagaaggatcttaaaggtatatatgggaagcttttaagaggtagagaaaccaactgggtatatattttcttttatttgatttcaactagcaagagactaagactgatgtttgtttgtttgttttaccttcaaagtcttagtcttaaattgacaagggcacaaaaaaagtgaaattaaaataattttaacaaaagggaaagcatttgacagtgtttaaaagacagacaaatcaagcaaaactcaatgtggcttaaggtaaaaaatacaactaggtattaaacaatttgtaaaaacttacaaagaaaatttagctttcaagaaaaattaggcagatttccttctgccaaagtgacaggtcctgaggaaaaaaaacacaacctctacaagaccaagcacagctcaagggtcagggccccgtcctagtcatctttttattattcaatatccatcacagtggctgggcaaacaacaggcatcaataaatgtttactaactgaatgtgtattataaggtataatcggtataactgatatagctcaaatctaatcatgaaagcttctttaaagtaggataaaaagagcacaatcagcggtattccagaaggtaggcctaaatccagttatatttttctaatcgttgaccagtggttataaagactttctgagcttctttttaaagcaatgaaactctttccaaaagaaaccccatgcagttcttcagtacagaataaatatgccactaagtcagtgagaactccaacagcctcccctaagccagcccccaaggtgtctctgtggaacctactggaaaaaatattactcatcttagaaatgtgatagaaagcatggccattcggttctcaggtcatcattcctagaaaattaacagtattgtgaagaataaatcctaagtaatgttgctaatttaaataaagacaaaaattcaacaaagaggggattctatcacttagaaaaatgaaaaccacacctataaatggggggaggggcagaaaacaaaaaaaaaatcaggccacagtagataaaatacaaaaaacatcatctcgttaaaaagcatcaaacacattcacacaaatgtaattacaaccaggaagtaaactgctcaacaggtataactgctcaataggtgttttcaaagagttgagtcccaatttcatactgtacagaaaaatcgcatcagaactgtagagatgcgctccactactgaaacagcatagtaggcactgcttgacctaacacagtaatgcaagagtaaccaccaagatcaggaccttctaccactttcagagttgttttctgcccctacaactgttccctaacaccattacaagttctcaagtaagaaaaagaagggcagaggctccactgagtatctcctacaggcctgatagtggtattacctaggacatttactctgctcacaagatgggtagtggaagacataattactggacagcacaaagtctggaagcaagcagcagggcactaaaacagtgagagcttacacaacaaaagcttgttaaattaagtagtactgatgtggtgcaaatgaaatttttacagcaaaggttgaggaaggagatatgttagtgagaatcacatgaagcagactatcacaaaataaggccaccttcaaaatgttatgaactgtagaaccattctgatcttcaagtttggatttgtatagaggtttctgtataaagcattaatacctaatcaggagtttcctttagtgtgaacctttttgcatttgatgctattctctttgccaggaatgcttatctcccctggctcctcacttggcttgcttctttaatgtcaggtgttagctcatgcatcctttccttagaggctttccttgatgtcctacctgaagcatcccatctgttattctccagtacagtaccctgtttatctccttcatagacaagtaagataattaagggttagtgtaactgctgtctcagcaaaggcaggaactgtagttgtcttgttcacctttacccaaagactaagaaaagttcctggtacaaacaggtgaacaataaatatttgttgaatgaataaaaaattactataccaaatttacatgaacacatacatatacacacaaatataggaaaatggggagtacccaatagaaaaccaccaaatgttgaaagtattgaaaatgatacctatagagacaggtggatatgatttcaaagaacaagtaccaaagacagcttcaaaaatatgaaaatttatgaaaagacgaccaggagtggttattttccatttctactaagatgcaaacaagaagaaatgtttaaactgcaatgagtcaacatcagacataataattatttgctgcagaatgaactagcaacagagtttcggaaatctcctctcactacagagcatgaaatattgtcaatcacaaaaccaggatcagttaagaacagctcagactgcaggtaacttataagctaaaaaacttgctaaataaatggcttttcccccaatttttaaaattctgaattcataattatgtgtagaataacaatcaatttataaactgaatacaacatactttaaaaacagatggcccatatctgctgatcctacctcagcatcacttttctaggtattttgcagaaacaattacatttacaaaaggcccatttcataatgcaatctggttactaaaccaaatcaaactactcgaagagcagaaggtctgctgttgaaatattgtaaaatacctttggaaaaacggtatttatagattagcttttttaaaaagggataaatatgtggaagtaattctagcatatccctgaaaataattatactgccacctatgcattttttatgaggtggaaggataaatcaacagactgctagattatacaagccaattattcctgttgaaatttgggcataagacaaagggactttctccatatgaattcttactgtatcccagaattaactggtgccagcagtatcaatgcaactattactggtgatgatgtcatgttatgctgttttgattatgaggacaaaaatgggaatggaaaaaagaggcttggaaaggttttcagtatggtttccttataataagatttagcagttaaaaaaaaaaacaaaaaaaaacaaaaaaccacaaaaagaatgactgtttaagccccactgaacacattaaggtcaaggatttcaaaagttaatccacttttcttcccccaagagtttatttttggtaaaaggcagaaaaattagtttttctacaggaaaatctgcttctaaataatttgaaaatcttgatatatattatatattaaaaaagacacacaaaaataacagagaagtgggaataacagattaggtactgcaactttataaaggtttgcctagatcaagaagcagcgcacacacacacctcatctatgcaaactaaaaatgtatataaacagcacaatactgtgatactggatcatgatacattacctgtacacataactactactgttattaataaacctttgggacactcagttttatgcccaataagacatcattaagtctttaaaatcttctcttcctctttaatgggagagtatttctagacactaattttcccatctaatattcaaatataggaaacagattccacaaggtgctttaattgatgagacctcaagtgctgttttctctcttgaacttttggatagtaaacagtccatagggaccacacacaatgctatgacagaagagttgttacattaagtcttttcatgggacttgattggtgaagctttatgacatgcttgagcaacgcactgaaggggatcccatctgagttaatactttgtccaaccactgtagaggtccattcagatgaagttcaatccagcaaggagtacttgttaccgtctgccttcggtattctgctccccaccctttcacaaaactcattcttatggtgcacattctagttagctgatagacggcttcaaaaccctgattaacagactgagccagaagagcagcaaattcctggttgttgaagatcttcagattacagcctggtggaattttacacactgttgcagggtgccagccatatctctgattacaattggggctctgcacaaagattgcactatcacttaggcactcagcaaaaacttccccacctatgtagtataagcgcactcctcttcctatatgccttcttgtcatttctaccgtggcatttcggttaacattggagagtaaacctaagcagaacctctctgaatttgatgggtctgtaaagccatctacagtgagtgagggctgtgatgcatggaaggtttctccaaccctctgatttaattcataatatgctatcgaacaccaaaatgcaggttctgagtaagtaactggctgtaaatccaagctatgattaacaggggaaagagtagtaggagatagttctgctggagagcctgtgtccatactttgattcaactgttggtcacttgtttctccatcttcactgatatatccaggaggtggcgtttctggaatataattactctgtggctcaattcctgctgggaagttagtgttttctggaatggagtgagtatagtcatccagaggcggaagttctgttaggatctcggtgtgtcggggcactaatactggaggcaaaactggtgtctcaactctctgatagtggtaagggtttacacatacttcatcctttttaagattaaaagcatattcgcagttttcaattgccttgagttcatgatgactgtgaagatcaggccagcgccataatcggcaatatataacatgtggcaatccttttcgatgggatacctggagacgaccatcaagagaccttggtatggtaacacatttagtattacagttttgagtggtgatggctttctcaagctcatctaatcgtcctgttttctttagcttcttcaccagacttttcactgctttctcacaccacttttcttcctgcccattctgctctcctccgcctgctcctccagacccaccagctgacttcttccatcccagcagtctcttcacaactggcggcgtgaatggcaagatggacgacatgttcttaccaaaggcagcaagccacgctaggaaaacagcctcttgtatcgaacctcccggcggctggcgggctgctggctggcgagctgcttctccgccgccgcggccgcgcgggtagacccgcct

SEQ ID NO: 15520 - RNA, 6354 nt, Homo sapiens
  source 1..6354: mol_type = other RNA
gctgggattacaggcatgagccactgtacttggccaaaaattttaaataaacaacatgaggattctagctctcactacagagtagttcttcttttgtttttttgtttttgtttttgtttttgtttttttgaaatggagtttaactcttgttgcccaggctggagtgcaatggcgcgatctcggctcaaccgcaacctctgcctcaggggttcaagcggttctcctgcctcagcctcctgactagctgggattacaggcatgtgccacaacgcacagctaatttttttgtagttttaatagagatggggtttctccatgttggtcaggctggtctcaagctactaacctcaggtaatccgtcctccttggcctcccaaagtgctgggaagagtatagttcttcttaatccaacaaaaaagtattttactcacaacaaatataaattgcccccatcaacaaatgtatgtaatatcaaggataacgtgtacaaacaaagttgcactaacaaagtaaaaatttatcccacatacatgaaagcacagtgctaagttctggggaagcagacagtttctgctttcagggagcttccagtctggtagagatttacacagaaggcagattaaagagaatgatgatctcctttgttcagagataaaaaggaagcaaaaaagcaggtcaaatcaaagatgatctgcagaatacattaaccctacactgaaatcatggacctactccagtaattaaggctgcagaggtggggctgggtggatgaaaacatcagaagacaattacagcatgagatattgattgattgattgattgattgattgagacagggtctcactttgccacccaggctagagtacagtgacaccaacttggctcactgcagcctccacctcctggagctcaagtgatcttcccacctcagccccctaattagctgggactatatgtgtgtgtcaccacacccagctaatttgtgtattttttgtagagatagggattcgccaggttgcccaggctggtctcaaactcctgagctgaagtgatccgcctgccttggcctcccaaagtgctaggattacaggtgtgagccactgtgcccagctgagatttattttttctttattaatcagcaaaatagataccctatttatttcaagatacgattaactaatttttttgctaacaaccatttcctaaggtaaaatgaggcagaaagaaaaggagtatgacactatattcactgagtcttcgattttcttctaacagcctgtatcagtggctctcaactgggggcaattttgcctctcagaatggcaatgtttgaagacatttttggccataacaactagggggatggtacttgtagctagagggcagaggtcagggatattgctaaacatcctataaagtacagcatagcatcccaaaataaagatttatccagtccaaaatgtcaatgctgagattaggaaaccatgccatggttggataaaaaagatgaaaaaatcagtatgtctatagtataaaagcaattagtagcactttaagatagattgaacaggaacattctcttcctttatcagacagttgcagaccttctaaaaatatctgatagatctataatgggaaaataaaacatgctgagaagtagcacaaatttttctaaacttcaaatattagcatacaaatgaaaaacaaacttggaagacagaaaggacaagccaggcatggtggctcacgcctgtaatcctagcactttgggaggccgaggtgggtgggtcacaaggtcaggagtttgagaccagcctggccaacatggtaaaaccctgtctctactaaaaatacaaaaatcagctgggcgtagtgacgtatacctgaaatcccagctacttgggaggctgaggcaggaggactgcttgagcccaggagagggaggttgcagtgagccgagatcatgccactgcactccagcctgggcaacagagcatgacaatgtctcaaaaaaaaaaaaaaaaaagaaaggacaattttgttgctcaattgatcttatcaactgtttctgcaaccacaaaagcaaatgtggtcatgtttctgattttagttaagtccaaaaatatttattaaagtcttatcactaaaaatggccacaaatattaaaaataaaatattagtttttagattcacagaagaaaaaaatagccactgacacttgaggagatgctcaattccgatgagggacattcaaagttactttccaacattatctgaaaagtattgatcctttttttttttttttgagacgcagtgtcgctctgttgcccaggctacagtgcagtggcatgatcttggctcactgcaacttccaccccccagattcaagcaattctcctgcctcagcctcccgagtagctgggattacaggcttgcaccaccacatccagctaatttttgtatttttagtggagacagggtttcaccgtgtttgaccaggttggactcctgacctcaaatgatccgcccacttcagcctgccaaagtgctgggattacaggcatgagccactgcacacagcccaaagtatttatcctttattttgtggttatatgttgggaaagaagaacgtggaaaagaagtgaactaacaaattttcaggtattaatattacaattcagtacattctgacaaaaagaattatttcctatgaaattacacccattggctgggtgcagtggttcacggctgcaatcccagcactttgggaggccaaggtgggaggatcacttgaggccaggaattaaagactaccctgggcaacacagcaagaccctgtctctacaaaaaaagaaaaagaaaaaaaaattacacccactgagaaacagaatgtgtaacagtaaaacaacagagcagcttccatgtgattttgataggaaagctttaattggtgactaagctttgtaaaaaggatgtaaacaggggaaagaatgaaaagaataagatttatctacataatgaagtttgactttttacagtaaataaaatacctatttattaatatttccaaatattaattagatttaataatactatatatttgttacaatgccttcatcagaaaatttaataattaagaagatacttgaagttcattcaaatggcacttgcagaaatgcaacttaatttctagttctatcatatctgtctccaaaatggacatatatgacagcaaaaacaaaattctctataaatctctccattagttacattactatgtaactaaaatagctagttctataataaaaggattttatgtgccaaatcctgaccaagagagaaataaagtcattattgctgcaaatccaaatggaacctaacccaaatgtagggaggggcaaataaagtgaaaacatgttggaaggtggggtcaactgccttaggacaattctacatccagcttgacactactcacgacttactcctcctcactgtttcttccaagaaagtctaagcatgtgaaactgtccttgttgctccctgtggatctctggctgagtggctaaagggcaatcctgagcatagacacactctcctcccttctatcagctgtcccccacacatactcacagggatgagtagactgaacaaacatcaaaaagacgcaggaacaaataaaataccccaataaaggcaattcttaagtggtcaataaattagggcacttcttcaaattaagctctgtcaattaggcacttaataaaaacaaaagacatttatacaagcatctaaataacaaagaaagataaagaacaagagaaagacaagatttatgttaactaccagcatgttatacttcagccagaagtttttgaaagaaacgttatttgagaaggaaaataagtagtatttttctgtttcttaaaaatcaatattctttctagttcattaactaaaattagtttttcagtgttttcaacatagaaagaatgctcagattttggttgaacaaggaaaaattaaggcagtgtctttaagaccagtaaaggaaagcattaactatctcataagcttatctgagagggacatattaagctcatatttggatataatattaggaaattatggctttaaacataaaatattaatgtttcaaaattccacattttctcagttattctttctttttagctatatgtacttcaaatagcccacttaaagaattaaagaaatacgtttcacataattttggaacaatatgtgcatggtacttgacccagaactattagcttggatggtaaatcattatgttcctatgtaccactgacccagtataaaaaggaagaggacccataactgtcaaaatgtggttggaaatgactaatgtcctttggaatttgctacaaaatagaagatataaagttttgaggtattgctgccttaccatggtttaggggaaaaaaataagagttttttgttccgttttgtttttttaaaagcaatgcttcttaagttatgaagcttatttaaaattttctcctcttagtcattgtcatatgggttatccctgagcttcatctcatctgcacgtcacataaaccagctacctatggttttgatcatttcatttagtgttatgtcttgttataccaattcatggagcgtttcactgctttggcccagttttccagactcatttcatattcttgacatttcttctgtggcttgaaaaccacttcactttgtctcagtttctttagttcctccttgtcagtccaaaacccaacagcaaggccagctagagaagctgcacccaggcatgacatgtcaatgtcggcaggtctgtctatattctcattaatcaggtctgaagtcatctgcatgacaaaaccattcttacaaactcctccatctgcccggatttttcttacaggaatatgaatctctttcttcatcatctcatataactgtttgtttctgaaagctattgactccaatattgctcgtacaagatggtatttactggtagaaggcttcaaacccataaaagaggcacatgcccaggggtcatttaatggagcctgtaatccactaaaagatggaacaaaacaaactccttcagaatcctccaaacttttggccattttttcagtctcagcagcatctgtgaaaaggtctaactgctgagcccattttatggcagtaccagtgtctcctgcattgctttcagctaagcatacgacttcttgcccaatcttccacccaattaatggataaaagcctccagtagtctgttgaaggctatttccagtgttaatatccaaaaatgtcccagttcccatggttaatttcacatcacctgtctggaagcagcactctccaaacatggctgattgctggtcagcaaccaaggcaactattggtataggcacaccaaatatctcttcatccactgatccaaaattgtggcttgtgtccctcacaggaggtaggagagaaagtggtatcgaaattagagaggtaatcatcccactccaacacatcttatatgggtcaaaaagtccagttgtactagcatttgaaaaatctgtggcatatacagaaccttttgtgagcttatataacaaccaggtatcaatagtcccaaagcagcaattttcttcttcaactgccttttgcacctcagtcaagttctgtaaaatccagaccaatctcaaagaagtctgctgggttgtgaaagtgaacaaactggctgtaaaaagtcgtttacttctagtgaaaaagtgaagcactcggcaagaactgtgaaatatcttcataagaagagaattattccaagattttacaagttcaacagctcttaagtcttgccaacttataaagttgtgaaaatgatttcctgttttcttgttccacgtaataaaagttgctctctgtgttgaaatgccaagaccaacaatttgattcatctgtattcctgcagctttgactgcttcttttattacggcaacaaattgaatccaaagaacatcaggatcaatttctacccagccaatttgaggataaagattttctaccttctgcacgctggagccgcagacccgcgccgcccggtcatagacgtggcagcggatcacagaactgcccacatccagccccagcacgaagccggggtaccgcggctcctgcgctctctgctccgggtccgtgagcagccccgacatcccgatcccgcacgcctctccgctacagccgcctacccagagggcgcgctacaaatcccaatgctccagagtccccgggcggcccaacccgggccccaacccggctcagccggagagcctagagaggcct

SEQ ID NO: 15521 - RNA, 7437 nt, Homo sapiens
  source 1..7437: mol_type = other RNA
gctgggattacaggcatgagccactgtacttggccaaaaattttaaataaacaacatgaggattctagctctcactacagagtagttcttcttttgtttttttgtttttgtttttgtttttgtttttttgaaatggagtttaactcttgttgcccaggctggagtgcaatggcgcgatctcggctcaaccgcaacctctgcctcaggggttcaagcggttctcctgcctcagcctcctgactagctgggattacaggcatgtgccacaacgcacagctaatttttttgtagttttaatagagatggggtttctccatgttggtcaggctggtctcaagctactaacctcaggtaatccgtcctccttggcctcccaaagtgctgggaagagtatagttcttcttaatccaacaaaaaagtattttactcacaacaaatataaattgcccccatcaacaaatgtatgtaatatcaaggataacgtgtacaaacaaagttgcactaacaaagtaaaaatttatcccacatacatgaaagcacagtgctaagttctggggaagcagacagtttctgctttcagggagcttccagtctggtagagatttacacagaaggcagattaaagagaatgatgatctcctttgttcagagataaaaaggaagcaaaaaagcaggtcaaatcaaagatgatctgcagaatacattaaccctacactgaaatcatggacctactccagtaattaaggctgcagaggtggggctgggtggatgaaaacatcagaagacaattacagcatgagatattgattgattgattgattgattgattgagacagggtctcactttgccacccaggctagagtacagtgacaccaacttggctcactgcagcctccacctcctggagctcaagtgatcttcccacctcagccccctaattagctgggactatatgtgtgtgtcaccacacccagctaatttgtgtattttttgtagagatagggattcgccaggttgcccaggctggtctcaaactcctgagctgaagtgatccgcctgccttggcctcccaaagtgctaggattacaggtgtgagccactgtgcccagctgagatttattttttctttattaatcagcaaaatagataccctatttatttcaagatacgattaactaatttttttgctaacaaccatttcctaaggtaaaatgaggcagaaagaaaaggagtatgacactatattcactgagtcttcgattttcttctaacagcctgtatcagtggctctcaactgggggcaattttgcctctcagaatggcaatgtttgaagacatttttggccataacaactagggggatggtacttgtagctagagggcagaggtcagggatattgctaaacatcctataaagtacagcatagcatcccaaaataaagatttatccagtccaaaatgtcaatgctgagattaggaaaccatgccatggttggataaaaaagatgaaaaaatcagtatgtctatagtataaaagcaattagtagcactttaagatagattgaacaggaacattctcttcctttatcagacagttgcagaccttctaaaaatatctgatagatctataatgggaaaataaaacatgctgagaagtagcacaaatttttctaaacttcaaatattagcatacaaatgaaaaacaaacttggaagacagaaaggacaagccaggcatggtggctcacgcctgtaatcctagcactttgggaggccgaggtgggtgggtcacaaggtcaggagtttgagaccagcctggccaacatggtaaaaccctgtctctactaaaaatacaaaaatcagctgggcgtagtgacgtatacctgaaatcccagctacttgggaggctgaggcaggaggactgcttgagcccaggagagggaggttgcagtgagccgagatcatgccactgcactccagcctgggcaacagagcatgacaatgtctcaaaaaaaaaaaaaaaaaagaaaggacaattttgttgctcaattgatcttatcaactgtttctgcaaccacaaaagcaaatgtggtcatgtttctgattttagttaagtccaaaaatatttattaaagtcttatcactaaaaatggccacaaatattaaaaataaaatattagtttttagattcacagaagaaaaaaatagccactgacacttgaggagatgctcaattccgatgagggacattcaaagttactttccaacattatctgaaaagtattgatcctttttttttttttttgagacgcagtgtcgctctgttgcccaggctacagtgcagtggcatgatcttggctcactgcaacttccaccccccagattcaagcaattctcctgcctcagcctcccgagtagctgggattacaggcttgcaccaccacatccagctaatttttgtatttttagtggagacagggtttcaccgtgtttgaccaggttggactcctgacctcaaatgatccgcccacttcagcctgccaaagtgctgggattacaggcatgagccactgcacacagcccaaagtatttatcctttattttgtggttatatgttgggaaagaagaacgtggaaaagaagtgaactaacaaattttcaggtattaatattacaattcagtacattctgacaaaaagaattatttcctatgaaattacacccattggctgggtgcagtggttcacggctgcaatcccagcactttgggaggccaaggtgggaggatcacttgaggccaggaattaaagactaccctgggcaacacagcaagaccctgtctctacaaaaaaagaaaaagaaaaaaaaattacacccactgagaaacagaatgtgtaacagtaaaacaacagagcagcttccatgtgattttgataggaaagctttaattggtgactaagctttgtaaaaaggatgtaaacaggggaaagaatgaaaagaataagatttatctacataatgaagtttgactttttacagtaaataaaatacctatttattaatatttccaaatattaattagatttaataatactatatatttgttacaatgccttcatcagaaaatttaataattaagaagatacttgaagttcattcaaatggcacttgcagaaatgcaacttaatttctagttctatcatatctgtctccaaaatggacatatatgacagcaaaaacaaaattctctataaatctctccattagttacattactatgtaactaaaatagctagttctataataaaaggattttatgtgccaaatcctgaccaagagagaaataaagtcattattgctgcaaatccaaatggaacctaacccaaatgtagggaggggcaaataaagtgaaaacatgttggaaggtggggtcaactgccttaggacaattctacatccagcttgacactactcacgacttactcctcctcactgtttcttccaagaaagtctaagcatgtgaaactgtccttgttgctccctgtggatctctggctgagtggctaaagggcaatcctgagcatagacacactctcctcccttctatcagctgtcccccacacatactcacagggatgagtagactgaacaaacatcaaaaagacgcaggaacaaataaaataccccaataaaggcaattcttaagtggtcaataaattagggcacttcttcaaattaagctctgtcaattaggcacttaataaaaacaaaagacatttatacaagcatctaaataacaaagaaagataaagaacaagagaaagacaagatttatgttaactaccagcatgttatacttcagccagaagtttttgaaagaaacgttatttgagaaggaaaataagtagtatttttctgtttcttaaaaatcaatattctttctagttcattaactaaaattagtttttcagtgttttcaacatagaaagaatgctcagattttggttgaacaaggaaaaattaaggcagtgtctttaagaccagtaaaggaaagcattaactatctcataagcttatctgagagggacatattaagctcatatttggatataatattaggaaattatggctttaaacataaaatattaatgtttcaaaattccacattttctcagttattctttctttttagctatatgtacttcaaatagcccacttaaagaattaaagaaatacgtttcacataattttggaacaatatgtgcatggtacttgacccagaactattagcttggatggtaaatcattatgttcctatgtaccactgacccagtataaaaaggaagaggacccataactgtcaaaatgtggttggaaatgactaatgtcctttggaatttgctacaaaatagaagatataaagttttgaggtattgctgccttaccatggtttaggggaaaaaaataagagttttttgttccgttttgtttttttaaaagcaatgcttcttaagttatgaagcttatttaaaattttctcctcttagtcattgtcatatgggttatccctgagcttcatctcatctgcacgtcacataaaccagctacctatggttttgatcatttcatttagtgttatgtcttgttataccaattcatggagcgtttcactgctttggcccagttttccagactcatttcatattcttgacatttcttctgtggcttgaaaaccacttcactttgtctcagtttctttagttcctccttgtcagtccaaaacccaacagcaaggccagctagagaagctgcacccaggcatgacatgtcaatgtcggcaggtctgtctatattctcattaatcaggtctgaagtcatctgcatgacaaaaccattcttacaaactcctccatctgcccggatttttcttacaggaatatgaatctctttcttcatcatctcatataactgtttgtttctgaaagctattgactccaatattgctcgtacaagatggtatttactggtagaaggcttcaaacccataaaagaggcacatgcccaggggtcatttaatggagcctgtaatccactaaaagatggaacaaaacaaactccttcagaatcctccaaacttttggccattttttcagtctcagcagcatctgtgaaaaggtctaactgctgagcccattttatggcagtaccagtgtctcctgcattgctttcagctaagcatacgacttcttgcccaatcttccacccaattaatggataaaagcctccagtagtctgttgaaggctatttccagtgttaatatccaaaaatgtcccagttcccatggttaatttcacatcacctgtctggaagcagcactctccaaacatggctgattgctggtcagcaacctatagtcctagctactcaggaggctgaggcagaagagtcacttgaacccgagaggcggaggtcacagtgagccatcggtgagatcatgccattgcactccagtctgggagacaagagtgaaactccatctcaaaaacaacaacaacaacaacaactcatttaaagaaccctctgtcactaattggtaactcttccagccataccttaatctaaccctgcacctatgcctagattgaataagaccgatcctctctaaatgataatgattttgtaacttggaaattaaattccctttccctcagctgctcccccagctactgtggagactgcacatcttgcaacaggtggtctctacctcctgcttaagctgccacaggaaatcaaaggcaatgtgaaaggactcttaaaaatcaaaaacaggcttggcacagtgactcatgcctgtagtcccagcactttgggaggcaaaggtggcagaaggccccagtctaggagttcgagatcagccaggggaacacagcaaaatcctatgtctaccaaaaatacaaaaaattagccaggtgtcgtggcacacacctgtggtcttggctacttgggaggctggggtggaagaatcacctgagcccaggaagccgaggctgcagtgaggcatgattataccactgcactccagcctgagtgacagagtgagaccctgtctcaaaaaaaaaaaaaaaaatcaaaaatggcaaatatttcattattctacaaacttatttactggtagatgatggctaaggactttattaaatgtacatacaactttctctgctagtttaagttgccctaacactgtttgtggttacacattatcaaacagaacataaatattcgccccatcactgtgttttgtctcagagtaccaaatgtaaactaaataccactcagaattaaaaaaaattttttttaatttaagttttctgataaacaatatacaagcaagtcagaaaaggttataaagtacttccatgatagaatactggctcaatggtccccttcccaaaaatatagcagatattctggtcatatccagggacctttaacaaggcaactattggtataggcacaccaaatatctcttcatccactgatccaaaattgtggcttgtgtccctcacaggaggtaggagagaaagtggtatcgaaattagagaggtaatcatcccactccaacacatcttatatgggtcaaaaagtccagttgtactagcatttgaaaaatctgtggcatatacagaaccttttgtgagcttatataacaaccaggtatcaatagtcccaaagcagcaattttcttcttcaactgccttttgcacctcagtcaagttctgtaaaatccagaccaatctcaaagaagtctgctgggttgtgaaagtgaacaaactggctgtaaaaagtcgtttacttctagtgaaaaagtgaagcactcggcaagaactgtgaaatatcttcataagaagagaattattccaagattttacaagttcaacagctcttaagtcttgccaacttataaagttgtgaaaatgatttcctgttttcttgttccacgtaataaaagttgctctctgtgttgaaatgccaagaccaacaatttgattcatctgtattcctgcagctttgactgcttcttttattacggcaacaaattgaatccaaagaacatcaggatcaatttctacccagccaatttgaggataaagattttctaccttctgcacgctggagccgcagacccgcgccgcccggtcatagacgtggcagcggatcacagaactgcccacatccagccccagcacgaagccggggtaccgcggctcctgcgctctctgctccgggtccgtgagcagccccgacatcccgatcccgcacgcctctccgctacagccgcctacccagagggcgcgctacaaatcccaatgctccagagtccccgggcggcccaacccgggccccaacccggctcagccggagagcctagagaggcct

SEQ ID NO: 15522 - RNA, 3052 nt, Homo sapiens
  source 1..3052: mol_type = other RNA
gctgggattacaggcatgagccactgtatccagctaaaaactaaaataattaaatagcagtacttttacatgttgggtgattgtgggaattgttaaccttaaggagcagaataacacacttttagctaagtcttgatgaactatagtggagttttcaaattaaatcattcaaggagtcacatgaggtttacttgtgattttccagacattgaaaagaaaatcttttttcataacagatacttgttgctttgaggaatctgcattttaagaatattgtgcactgtgatttaaagccagaaaatgtgctgcttgcatcagcagagccatttcctcaggtgagatattctccagaaccttttaaatgattctggcaacattttcaaagcacccacataataaaaggcagtgtactaagtactgttggttaaaaatgcataccaccttacaaaaatagtttttagcctgtaactaccagtgaggattaataactaaatgaattcagatgttattagttatactgtttatattcaagattttttaagatttaactgcacatagattctgcaattcacctctccccaggggctgggaacgaagtgagcaagtatcaaccttggttggtgcatggtacttaggataaatacctcataaataaaacaaatggggtgttactggaaatgggagatagattttggttgaggcaggcagccacctcctttttctatgtagagtattgtattcaaacaacctacataaaataacatttctcatcaccacacatacacacaatggcatcgtgcttctgtgtcctggctacatgtagcactctctgatttttcttaattcagttgagttttttttttttccaagtgttcatcttgatccactaaatttattgcatgacctatgaaatggatcataacccaaattctgaaacaaccatcctgagaaataagtggtggtggtggtaccctgcagccattttccataattggcaaggatgattcctccgatcagctcaaatatctgttgccaaactattgtttatatacatttgaaacatgtacatttagacaaatggcaagactaaggacaacagataggtgttttcacttggtaaatataactcaaattgtcttttcaaataaaaagatatattaaaaatcgttcagcttttaaagtagtaatcatattctttttatgtttatgtggttaaaagtgattccctatcattttgaggtcgaaagggttgcctgatagttggtgcaatgttttaaataaactgcttccatatattatctcatttgatcttcaaaatagtagacaaaagatgcacactcctactggtaacattaaaactcccactttctgacctctattttagtgatccacagtgttccaatgagaagcaaagggaaaataatgtgatttacttgatacgctttttatgctcaagtgttagccatggctccacttctttaatcagttgccaaacttccaagtcatctttaccttatcaagatgttagctgaaatctggcatttaacaacaaaaaaagagtttgtatttcttcaggctcagtattcgtactcttcaaagacactgcagtatatgaaatgtgtttcctttattttgatttcttgggccgactgaagggtaaaatgtccaagctgaaatatcactgccaagcaagttcactaaacccagctacaacggatgcaaagggttttgactgacgtgcattcctctgatatcttccaccttgaagtctctgatgaggtagcaaggcaaaaaagttaaatctctctcccatcttctttggattcattaacatatcatatccttgaagtaactgctgcctcactgatggctcatttgatttatctaaaagaaccttcagccggacatcaatacccatattttttaaaaatgtgtgttgttttattgggcccagagaggctacttttccctgtgccattcttcgcaaataactgaagtccacatcagctgttagatctgctgttcctggggcaattaagacatcatgaagcttgtggtcgcaaaaccctctgaaggtatctgtctttgttccatcatgaccataatcagcaaccagtgcagcacctccagttaatgcaatgcgttgagaaagttcctcgatgataacaccagcatcaggacacacttcaacatgatcccttgtttcgtcatgttgtatgaaggcttctgctggggtggcagaaggtgccaaaacaaacctcagtttatcagaaacctgtggatcaatgtcaacaaatacttctcgccatccctgtggtgttttctgaaatttatgcacaggaagaacatcaaaaaattcatgtgcaagataaaagctgtacccttttggaacatcgtgcagatctcggtaccaggaaattggaatcccagacttagtgacacctttcatatacactggggatccagcatttcgctctaacgggaccttctctttagtcagtgtcaatgcttgaatctcacttaatttttggcttacctctaccagatgtactgaaatgtcacaatttttcagcacagatccaagttgagtgaacaccctcaaaatatctcccacgagggttcccctacctgggcccagttccaccagctggaaagctgtgctttttccagtggccatccattcactaatgaaccatatacctagtagctccccaaagatttgacttatttcaggtgaagtaatgaaatctcctttttcgcctagcatgtcacggtacacataataacccttggctggattagtcaacacctccttcatgtactcggccacagtgatgggaccagtagactttattttgtacataagatgccgcagcatcggcgtcaccgggttttctgcaggctcattcccggagctgaagtatttccctctccaaataaaaggaatggctgcgcgcgccacggcacacaacggccccaaacctgacctcagcagtacactcatgctgaaattcgcaggctagctcgctccgccaggagctggggcttagac

SEQ ID NO: 15523 - RNA, 2233 nt, Homo sapiens
  source 1..2233: mol_type = other RNA
gctgggattacaggcatgagccactgtgaccagcctattattattttcaagacagggtctcactctgttgcccagcctggagtgcagtggtgtgatcatagctcaccgcagcctcaatctcctgggctgaagtgatccttctgtctcagcctccccaacagctgggagtatagcggtgcaacaccacacccagctttgctatttatttaaatgtcattctccaacacatatggggaatgacatatgcttcccattattacatggcaaaacatactccatatccagaaaaaatatttatatgacatatggcctagtattctaaatcaaggcaggatcttccaacaagagcaggagagagaagaaaacatttacattctataacatgattataagaattgagatagatgaaatgaaaaacaacatctttgaacaattacagttgacagaacagctttcccttattctacttgctttaaataactcatatctgtaaacttgaacaccaactctggctgatttaacagtcttaatcccttgattttccatactgaacatcacccaatatatagtgaagatcaaaggcgacttcttccaccaagctctgtgtccagctgtgtttctgaggtcatacgtgtcccctcacggacaccagatcagatacttcggtagtcagagccgcgggctacaaaggcggcagcttcccattccacagtgaagaaagaaattgttccaaaaaacccaaatatcaccatgaccaggagttgccagtgaaggagaaggtagttgctgtagaaaaatgccacggctgcgcaaatagactgaacaaacttgaagatggcaaatgctggggcgctgtcttcagaatacagaaagcccaagatactaagcagctgggtattaaagcagctgtctccaaggcccaacagaaaactgcagagaatggcaacttctggatttgatgtaagcactgctgtcagttcctttaacaggagcaatcggggcatctccaggcatgttgagaaatattagataaaaagctatgaagtgcaccaggatgcccaacagcacaactggatttctaccaaaacgattgttcttgctcagcaggccgaagaggcttccacctaaaatttctccaatgccgatgaaaatgccagaaagtccaataaggcttttctcttctgctccaaatttatttgtagcaccaatacaggttccatatacaccagagaagaaagttaattccagacctgtataagcagttgtaatactaagaaggagcatctccttggtgacacataacttaaaagacttttctggaaaaatgcaaaccctggggtgtcatcaatccaaagttaccagggaataggggaaaggcaaatgccgagttgttcctgaacagttcttgcatttcagatacagaaaatacttactaaaagcatctactgcctttgtcagattgttctgggcagactcgttgacttccatgtcctggtcatcagaagactcatcttctcctaggacattttcagaatctggtttccgaatgagaaagaatagaactgtccccacaaggctaatcaccgttagggcaataaacactgttcttcggtcactctctgatatctgagttttcccttgccaggcaaaatatatgtagagatttccaaagaacaagctagactgcagaagtgcccagaaaatcccactgtttctcccaatgctgtgctcatccgaattgattgtcaggcagtttccttgtgctgtccaaagcacagcagcagcaattccaatgaaaacagaggctgtgtagaaggaccacgggaaaggctggatgaaaacggcaatgtacatgctgtaaaataaaccactggcaaacatagagagttgaggtcctacaatggcaaccactgacggtgtaatcaaatttgaagcagagaacactccatagataatagccatgctggtatatccactgccgtgaaaatctgtcctatttaagctcctgatgacagtttgcgccacatttccacaagtttgaaaggcagtgaacataaacataaaggcaactcctaaaataatgatgttgaaaagctttttagattccggggacattttggctcagctctgccggaggcagcagcccagggcagtcagctctcctcggggcgaagccactgacaatccggcagttaggatactcctaagaagcgatccgagtacggaagagcac

SEQ ID NO: 15524 - RNA, 2173 nt, Homo sapiens
  source 1..2173: mol_type = other RNA
gctgggattacaggcatgagccactgtgaccagcctattattattttcaagacagggtctcactctgttgcccagcctggagtgcagtggtgtgatcatagctcaccgcagcctcaatctcctgggctgaagtgatccttctgtctcagcctccccaacagctgggagtatagcggtgcaacaccacacccagctttgctatttatttaaatgtcattctccaacacatatggggaatgacatatgcttcccattattacatggcaaaacatactccatatccagaaaaaatatttatatgacatatggcctagtattctaaatcaaggcaggatcttccaacaagagcaggagagagaagaaaacatttacattctataacatgattataagaattgagatagatgaaatgaaaaacaacatctttgaacaattacagttgacagaacagctttcccttattctacttgctttaaataactcatatctgtaaacttgaacaccaactctggctgatttaacagtcttaatcccttgattttccatactgaacatcacccaatatatagtgaagatcaaaggcgacttcttccaccaagctctgtgtccagctgtgtttctgaggtcatacgtgtcccctcacggacaccagatcagatacttcggtagtcagagccgcgggctacaaaggcggcagcttcccattccacagtgaagaaagaaattgttccaaaaaacccaaatatcaccatgaccaggagttgccagtgaaggagaaggtagttgctgtagaaaaatgccacggctgcgcaaatagactgaacaaacttgaagatggcaaatgctggggcgctgtcttcagaatacagaaagcccaagatactaagcagctgggtattaaagcagctgtctccaaggcccaacagaaaactgcagagaatggcaacttctggatttgatgtaagcactgctgtcagttcctttaacaggagcaatcggggcatctccaggcatgttgagaaatattagataaaaagctatgaagtgcaccaggatgcccaacagcacaactggatttctaccaaaacgattgttcttgctcagcaggccgaagaggcttccacctaaaatttctccaatgccgatgaaaatgccagaaagtccaataaggcttttctcttctgctccaaatttatttgtagcaccaatacaggttccatatacaccagagaagaaagttaattccagacctgtataagcagttgtaatactaagaaggagcatctccttggtgacacataacttaaaagactttttaaaagcatctactgcctttgtcagattgttctgggcagactcgttgacttccatgtcctggtcatcagaagactcatcttctcctaggacattttcagaatctggtttccgaatgagaaagaatagaactgtccccacaaggctaatcaccgttagggcaataaacactgttcttcggtcactctctagactgcagaagtgcccagaaaatcccactgtttctcccaatgctgtgctcatccgaattgattgtcaggcagtttccttgtgctgtccaaagcacagcagcagcaattccaatgaaaacagaggctgtgtagaaggaccacgggaaaggctggatgaaaacggcaatgtacatgctgtaaaataaaccactggcaaacatagagagttgaggtcctacaatggcaaccactgacggtgtaatcaaatttgaagcagagaacactccatagataatagccatgctggtatatccactgccgtgaaaatctgtcctatttaagctcctgatgacagtttgcgccacatttccacaagtttgaaaggcagtgaacataaacataaaggcaactcctaaaataatgatgttgaaaagctttttagattccggggacattttggctcagctctgccggaggcagcagcccagggcagtcagctctcctcggggcgaagccactgacaatcctggagaaagaaatgagatggtgagtggagaaggcagatgcaggagccaggcagccaagctgtcaacttccagttcctggatcggaaccccaggtttagggcgaagttctccccaccggcagttaggatactcctaagaagcgatccgagtacggaagagcac

SEQ ID NO: 15525 - RNA, 2590 nt, Homo sapiens
  source 1..2590: mol_type = other RNA
gctgggattacaggcatgagccactgtgaccagcctattattattttcaagacagggtctcactctgttgcccagcctggagtgcagtggtgtgatcatagctcaccgcagcctcaatctcctgggctgaagtgatccttctgtctcagcctccccaacagctgggagtatagcggtgcaacaccacacccagctttgctatttatttaaatgtcattctccaacacatatggggaatgacatatgcttcccattattacatggcaaaacatactccatatccagaaaaaatatttatatgacatatggcctagtattctaaatcaaggcaggatcttccaacaagagcaggagagagaagaaaacatttacattctataacatgattataagaattgagatagatgaaatgaaaaacaacatctttgaacaattacagttgacagaacagctttcccttattctacttgctttaaataactcatatctgtaaacttgaacaccaactctggctgatttaacagtcttaatcccttgattttccatactgaacatcacccaatatatagtgaagatcaaaggcgacttcttccaccaagctctgtgtccagctgtgtttctgaggtcatacgtgtcccctcacggacaccagatcagatacttcggtagtcagagccgcgggctacaaaggcggcagcttcccattccacagtgaagaaagaaattgttccaaaaaacccaaatatcaccatgaccaggagttgccagtgaaggagaaggtagttgctgtagaaaaatgccacggctgcgcaaatagactgaacaaacttgaagatggcaaatgctggggcgctgtcttcagaatacagaaagcccaagatactaagcagctgggtattaaagcagctgtctccaaggcccaacagaaaactgcagagaatggcaacttctttgctggatttgatgtaagcactgctgtcagttcctttaacaggagcaatcggggcatctccaggcatgttgagaaatattagataaaaagctatgaagtgcaccaggatgcccaacagcacaactggatttctaccaaaacgattgttcttgctcagcaggccgaagaggcttccacctaaaatttctccaatgccgatgaaaatgccagaaagtccaataaggcttttctcttctgctccaaatttatttgtagcaccaatacaggttccatatacaccagagaagaaagttaattccagacctgtataagcagttgtaatactaagaaggagcatctccttggtgacacataacttaaaagacttttctggaaaaatgcaaaccctggggtgtcatcaatccaaagttaccagggaataggggaaaggcaaatgccgagttgttcctgaacagttcttgcatttcagatacagaaaatacttactaaaagcatctactgcctttgtcagattgttctgggcagactcgttgacttccatgtcctggtcatcagaagactcatcttctcctaggacattttcagaatctggtttccgaatgagaaagaatagaactgtccccacaaggctaatcaccgttagggcaataaacactgttcttcggtcactctctagactgcagaagtgcccagaaaatcccactgtttctcccaatgctgtgctcatccgaattgattgtcaggcagtttccttgtgctgtccaaagcacagcagcagcaattccaatgaaaacagaggctgtgtagaaggaccacgggaaaggctggatgaaaacggcaatgtacatgctgtaaaataaaccactggcaaacatagagagttgaggtcctacaatggcaaccactgacggtgtaatcaaatttgaagcagagaacactccatagataatagccatgctggtatatccactgccgtgaaaatctgtcctatttaagctcctgatgacagtttgcgccacatttccacaagtttgaaaggcagtgaacataaacataaaggcaactcctaaaataatgatgttgaaaagctttttagattccggggacattttggctcagctctgccggaggcagcagcccagggcagtcagctctcctcggggcgaagccactgacaatccgcacctcgcccgacacgctgaggcgcgtcttcgagaagtacgggcgcgtcggcgacgtgtacatcccgcgggaccgctacaccaaggagtcccgcggcttcgccttcgttcgctttcacgacaagcgcgacgctgaggacgctatggatgccatggacggggccgtgctggacggccgcgagctgcgggtgcaaatggcgcgctacggccgccccccggactcacaccacagccgccggggaccgccaccccgcaggtacgggggcggtggctacggacgccggagccgcaggtaaacggggctgaggggaccgcgggaggcggggcggggcgcgcgggaggcccgggcgacctcacaaaggtccgcggcgaagcacgtggtgcgggcccggacggggcgggggtgcacgccgcgtctcgcgaccctccggccaccccgcgagcttccgccgtctgc

SEQ ID NO: 15526 - RNA, 2179 nt, Homo sapiens
  source 1..2179: mol_type = other RNA
gctgggattacaggcatgagccactgtgaccagcctattattattttcaagacagggtctcactctgttgcccagcctggagtgcagtggtgtgatcatagctcaccgcagcctcaatctcctgggctgaagtgatccttctgtctcagcctccccaacagctgggagtatagcggtgcaacaccacacccagctttgctatttatttaaatgtcattctccaacacatatggggaatgacatatgcttcccattattacatggcaaaacatactccatatccagaaaaaatatttatatgacatatggcctagtattctaaatcaaggcaggatcttccaacaagagcaggagagagaagaaaacatttacattctataacatgattataagaattgagatagatgaaatgaaaaacaacatctttgaacaattacagttgacagaacagctttcccttattctacttgctttaaataactcatatctgtaaacttgaacaccaactctggctgatttaacagtcttaatcccttgattttccatactgaacatcacccaatatatagtgaagatcaaaggcgacttcttccaccaagctctgtgtccagctgtgtttctgaggtcatacgtgtcccctcacggacaccagatcagatacttcggtagtcagagccgcgggctacaaaggcggcagcttcccattccacagtgaagaaagaaattgttccaaaaaacccaaatatcaccatgaccaggagttgccagtgaaggagaaggtagttgctgtagaaaaatgccacggctgcgcaaatagactgaacaaacttgaagatggcaaatgctggggcgctgtcttcagaatacagaaagcccaagatactaagcagctgggtattaaagcagctgtctccaaggcccaacagaaaactgcagagaatggcaacttctttgctggatttgatgtaagcactgctgtcagttcctttaacaggagcaatcggggcatctccaggcatgttgagaaatattagataaaaagctatgaagtgcaccaggatgcccaacagcacaactggatttctaccaaaacgattgttcttgctcagcaggccgaagaggcttccacctaaaatttctccaatgccgatgaaaatgccagaaagtccaataaggcttttctcttctgctccaaatttatttgtagcaccaatacaggttccatatacaccagagaagaaagttaattccagacctgtataagcagttgtaatactaagaaggagcatctccttggtgacacataacttaaaagacttttctggaaaaatgcaaaccctggggtgtcatcaatccaaagttaccagggaataggggaaaggcaaatgccgagttgttcctgaacagttcttgcatttcagatacagaaaatacttactaaaagcatctactgcctttgtcagattgttctgggcagactcgttgacttccatgtcctggtcatcagaagactcatcttctcctaggacattttcagaatctggtttccgaatgagaaagaatagaactgtccccacaaggctaatcaccgttagggcaataaacactgttcttcggtcactctctagactgcagaagtgcccagaaaatcccactgtttctcccaatgctgtgctcatccgaattgattgtcaggcagtttccttgtgctgtccaaagcacagcagcagcaattccaatgaaaacagaggctgtgtagaaggaccacgggaaaggctggatgaaaacggcaatgtacatgctgtaaaataaaccactggcaaacatagagagttgaggtcctacaatggcaaccactgacggtgtaatcaaatttgaagcagagaacactccatagataatagccatgctggtatatccactgccgtgaaaatctgtcctatttaagctcctgatgacagtttgcgccacatttccacaagtttgaaaggcagtgaacataaacataaaggcaactcctaaaataatgatgttgaaaagctttttagattccggggacattttggctcagctctgccggaggcagcagcccagggcagtcagctctcctcggggcgaagccactgacaatccggcagttaggatactcctaagaagcgatccgagtacggaagagcac

SEQ ID NO: 15527 - RNA, 2689 nt, Homo sapiens
  source 1..2689: mol_type = other RNA
gctgggattacaggcatgagccactgtgaccagcctattattattttcaagacagggtctcactctgttgcccagcctggagtgcagtggtgtgatcatagctcaccgcagcctcaatctcctgggctgaagtgatccttctgtctcagcctccccaacagctgggagtatagcggtgcaacaccacacccagctttgctatttatttaaatgtcattctccaacacatatggggaatgacatatgcttcccattattacatggcaaaacatactccatatccagaaaaaatatttatatgacatatggcctagtattctaaatcaaggcaggatcttccaacaagagcaggagagagaagaaaacatttacattctataacatgattataagaattgagatagatgaaatgaaaaacaacatctttgaacaattacagttgacagaacagctttcccttattctacttgctttaaataactcatatctgtaaacttgaacaccaactctggctgatttaacagtcttaatcccttgattttccatactgaacatcacccaatatatagtgaagatcaaaggcgacttcttccaccaagctctgtgtccagctgtgtttctgaggtcatacgtgtcccctcacggacaccagatcagatacttcggtagtcagagccgcgggctacaaaggcggcagcttcccattccacagtgaagaaagaaattgttccaaaaaacccaaatatcaccatgaccaggagttgccagtgaaggagaaggtagttgctgtagaaaaatgccacggctgcgcaaatagactgaacaaacttgaagatggcaaatgctggggcgctgtcttcagaatacagaaagcccaagatactaagcagctgggtattaaagcagctgtctccaaggcccaacagaaaactgcagagaatggcaacttctttgctggatttgatgtaagcactgctgtcagttcctttaacaggagcaatcggggcatctccaggcatgttgagaaatattagataaaaagctatgaagtgcaccaggatgcccaacagcacaactggatttctaccaaaacgattgttcttgctcagcaggccgaagaggcttccacctaaaatttctccaatgccgatgaaaatgccagaaagtccaataaggcttttctcttctgctccaaatttatttgtagcaccaatacaggttccatatacaccagagaagaaagttaattccagacctgtataagcagttgtaatactaagaaggagcatctccttggtgacacataacttaaaagacttttctggaaaaatgcaaaccctggggtgtcatcaatccaaagttaccagggaataggggaaaggcaaatgccgagttgttcctgaacagttcttgcatttcagatacagaaaatacttactaaaagcatctactgcctttgtcagattgttctgggcagactcgttgacttccatgtcctggtcatcagaagactcatcttctcctaggacattttcagaatctggtttccgaatgagaaagaatagaactgtccccacaaggctaatcaccgttagggcaataaacactgttcttcggtcactctctgatatctgagttttcccttgccaggcaaaatatatgtagagatttccaaagaacaagctagactgcagaagtgcccagaaaatcccactgtttctcccaatgctgtgctcatccgaattgattgtcaggcagtttccttgtgctgtccaaagcacagcagcagcaattccaatgaaaacagaggctgtgtagaaggaccacgggaaaggctggatgaaaacggcaatgtacatgctaaaatataacaggtcaaggtattacagtcaaacgatacctgtaaaataaaccactggcaaacatagagagttgaggtcctacaatggcaaccactgacggtgtaatcaaatttgaagcagagaacactccatagataatagccatgctggtatatccactgccgtgaaaatctgtcctatttaagctcctgatgacagtttgcgccacatttccacaagtttgaaaggcagtgaacataaacataaaggcaactcctaaaataatgatgttgaaaagctttttagattccggggacattttggctcagctctgccggaggcagcagcccagggcagtcagctctcctcggggcgaagccactgacaatccgcacctcgcccgacacgctgaggcgcgtcttcgagaagtacgggcgcgtcggcgacgtgtacatcccgcgggaccgctacaccaaggagtcccgcggcttcgccttcgttcgctttcacgacaagcgcgacgctgaggacgctatggatgccatggacggggccgtgctggacggccgcgagctgcgggtgcaaatggcgcgctacggccgccccccggactcacaccacagccgccggggaccgccaccccgcaggtacgggggcggtggctacggacgccggagccgcaggtaaacggggctgaggggaccgcgggaggcggggcggggcgcgcgggaggcccgggcgacctcacaaaggtccgcggcgaagcacgtggtgcgggcccggacggggcgggggtgcacgccgcgtctcgcgaccctccggccaccccgcgagcttccgccgtctgc

SEQ ID NO: 15528 - RNA, 2238 nt, Homo sapiens
  source 1..2238: mol_type = other RNA
gctgggattacaggcatgagccactgtgaccagcctattattattttcaagacagggtctcactctgttgcccagcctggagtgcagtggtgtgatcatagctcaccgcagcctcaatctcctgggctgaagtgatccttctgtctcagcctccccaacagctgggagtatagcggtgcaacaccacacccagctttgctatttatttaaatgtcattctccaacacatatggggaatgacatatgcttcccattattacatggcaaaacatactccatatccagaaaaaatatttatatgacatatggcctagtattctaaatcaaggcaggatcttccaacaagagcaggagagagaagaaaacatttacattctataacatgattataagaattgagatagatgaaatgaaaaacaacatctttgaacaattacagttgacagaacagctttcccttattctacttgctttaaataactcatatctgtaaacttgaacaccaactctggctgatttaacagtcttaatcccttgattttccatactgaacatcacccaatatatagtgaagatcaaaggcgacttcttccaccaagctctgtgtccagctgtgtttctgaggtcatacgtgtcccctcacggacaccagatcagatacttcggtagtcagagccgcgggctacaaaggcggcagcttcccattccacagtgaagaaagaaattgttccaaaaaacccaaatatcaccatgaccaggagttgccagtgaaggagaaggtagttgctgtagaaaaatgccacggctgcgcaaatagactgaacaaacttgaagatggcaaatgctggggcgctgtcttcagaatacagaaagcccaagatactaagcagctgggtattaaagcagctgtctccaaggcccaacagaaaactgcagagaatggcaacttctttgctggatttgatgtaagcactgctgtcagttcctttaacaggagcaatcggggcatctccaggcatgttgagaaatattagataaaaagctatgaagtgcaccaggatgcccaacagcacaactggatttctaccaaaacgattgttcttgctcagcaggccgaagaggcttccacctaaaatttctccaatgccgatgaaaatgccagaaagtccaataaggcttttctcttctgctccaaatttatttgtagcaccaatacaggttccatatacaccagagaagaaagttaattccagacctgtataagcagttgtaatactaagaaggagcatctccttggtgacacataacttaaaagacttttctggaaaaatgcaaaccctggggtgtcatcaatccaaagttaccagggaataggggaaaggcaaatgccgagttgttcctgaacagttcttgcatttcagatacagaaaatacttactaaaagcatctactgcctttgtcagattgttctgggcagactcgttgacttccatgtcctggtcatcagaagactcatcttctcctaggacattttcagaatctggtttccgaatgagaaagaatagaactgtccccacaaggctaatcaccgttagggcaataaacactgttcttcggtcactctctgatatctgagttttcccttgccaggcaaaatatatgtagagatttccaaagaacaagctagactgcagaagtgcccagaaaatcccactgtttctcccaatgctgtgctcatccgaattgattgtcaggcagtttccttgtgctgtccaaagcacagcagcagcaattccaatgaaaacagaggctgtgtagaaggaccacgggaaaggctggatgaaaacggcaatgtacatgctgtaaaataaaccactggcaaacatagagagttgaggtcctacaatggcaaccactgacggtgtaatcaaatttgaagcagagaacactccatagataatagccatgctggtatatccactgccgtgaaaatctgtcctatttaagctcctgatgacagtttgcgccacatttccacaagtttgaaaggcagtgaacataaacataaaggcaactcctaaaataatgatgttgaaaagctttttagattccggggacattttggctcagctctgccggaggcagcagcccagggcagtcagctctcctcggggcgaagccactgacaatccggcagttaggatactcctaagaagcgatccgagtacggaagagcac

SEQ ID NO: 15529 - RNA, 2354 nt, Homo sapiens
  source 1..2354: mol_type = other RNA
gctgggattacaggcatgagccactgtgaccagcctattattattttcaagacagggtctcactctgttgcccagcctggagtgcagtggtgtgatcatagctcaccgcagcctcaatctcctgggctgaagtgatccttctgtctcagcctccccaacagctgggagtatagcggtgcaacaccacacccagctttgctatttatttaaatgtcattctccaacacatatggggaatgacatatgcttcccattattacatggcaaaacatactccatatccagaaaaaatatttatatgacatatggcctagtattctaaatcaaggcaggatcttccaacaagagcaggagagagaagaaaacatttacattctataacatgattataagaattgagatagatgaaatgaaaaacaacatctttgaacaattacagttgacagaacagctttcccttattctacttgctttaaataactcatatctgtaaacttgaacaccaactctggctgatttaacagtcttaatcccttgattttccatactgaacatcacccaatatatagtgaagatcaaaggcgacttcttccaccaagctctgtgtccagctgtgtttctgaggtcatacgtgtcccctcacggacaccagatcagatacttcggtagtcagagccgcgggctacaaaggcggcagcttcccattccacagtgaagaaagaaattgttccaaaaaacccaaatatcaccatgaccaggagttgccagtgaaggagaaggtagttgctgtagaaaaatgccacggctgcgcaaatagactgaacaaacttgaagatggcaaatgctggggcgctgtcttcagaatacagaaagcccaagatactaagcagctgggtattaaagcagctgtctccaaggcccaacagaaaactgcagagaatggcaacttctttgctggatttgatgtaagcactgctgtcagttcctttaacaggagcaatcggggcatctccaggcatgttgagaaatattagataaaaagctatgaagtgcaccaggatgcccaacagcacaactggatttctaccaaaacgattgttcttgctcagcaggccgaagaggcttccacctaaaatttctccaatgccgatgaaaatgccagaaagtccaataaggcttttctcttctgctccaaatttatttgtagcaccaatacaggttccatatacaccagagaagaaagttaattccagacctgtataagcagttgtaatactaagaaggagcatctccttggtgacacataacttaaaagacttttctggaaaaatgcaaaccctggggtgtcatcaatccaaagttaccagggaataggggaaaggcaaatgccgagttgttcctgaacagttcttgcatttcagatacagaaaatacttactaaaagcatctactgcctttgtcagattgttctgggcagactcgttgacttccatgtcctggtcatcagaagactcatcttctcctaggacattttcagaatctggtttccgaatgagaaagaatagaactgtccccacaaggctaatcaccgttagggcaataaacactgttcttcggtcactctctgatatctgagttttcccttgccaggcaaaatatatgtagagatttccaaagaacaagctagactgcagaagtgcccagaaaatcccactgtttctcccaatgctgtgctcatccgaattgattgtcaggcagtttccttgtgctgtccaaagcacagcagcagcaattccaatgaaaacagaggctgtgtagaaggaccacgggaaaggctggatgaaaacggcaatgtacatgctgtaaaataaaccactggcaaacatagagagttgaggtcctacaatggcaaccactgacggtgtaatcaaatttgaagcagagaacactccatagataatagccatgctggtatatccactgccgtgaaaatctgtcctatttaagctcctgatgacagtttgcgccacatttccacaagtttgaaaggcagtgaacataaacataaaggcaactcctaaaataatgatgttgaaaagctttttagattccggggacattttggctcagctctgccggaggcagcagcccagggcagtcagctctcctcggggcgaagccactgacaatcctggagaaagaaatgagatggtgagtggagaaggcagatgcaggagccaggcagccaagctgtcaacttccagttcctggatcggaaccccaggtttagggcgaagttctccccaccggcagttaggatactcctaagaagcgatccgagtacggaagagcac

SEQ ID NO: 15530 - RNA, 2624 nt, Homo sapiens
  source 1..2624: mol_type = other RNA
gctgggattacaggcatgagccactgtgaccagcctattattattttcaagacagggtctcactctgttgcccagcctggagtgcagtggtgtgatcatagctcaccgcagcctcaatctcctgggctgaagtgatccttctgtctcagcctccccaacagctgggagtatagcggtgcaacaccacacccagctttgctatttatttaaatgtcattctccaacacatatggggaatgacatatgcttcccattattacatggcaaaacatactccatatccagaaaaaatatttatatgacatatggcctagtattctaaatcaaggcaggatcttccaacaagagcaggagagagaagaaaacatttacattctataacatgattataagaattgagatagatgaaatgaaaaacaacatctttgaacaattacagttgacagaacagctttcccttattctacttgctttaaataactcatatctgtaaacttgaacaccaactctggctgatttaacagtcttaatcccttgattttccatactgaacatcacccaatatatagtgaagatcaaaggcgacttcttccaccaagctctgtgtccagctgtgtttctgaggtcatacgtgtcccctcacggacaccagatcagatacttcggtagtcagagccgcgggctacaaaggcggcagcttcccattccacagtgaagaaagaaattgttccaaaaaacccaaatatcaccatgaccaggagttgccagtgaaggagaaggtagttgctgtagaaaaatgccacggctgcgcaaatagactgaacaaacttgaagatggcaaatgctggggcgctgtcttcagaatacagaaagcccaagatactaagcagctgggtattaaagcagctgtctccaaggcccaacagaaaactgcagagaatggcaacttctttgctggatttgatgtaagcactgctgtcagttcctttaacaggagcaatcggggcatctccaggcatgttgagaaatattagataaaaagctatgaagtgcaccaggatgcccaacagcacaactggatttctaccaaaacgattgttcttgctcagcaggccgaagaggcttccacctaaaatttctccaatgccgatgaaaatgccagaaagtccaataaggcttttctcttctgctccaaatttatttgtagcaccaatacaggttccatatacaccagagaagaaagttaattccagacctgtataagcagttgtaatactaagaaggagcatctccttggtgacacataacttaaaagacttttctggaaaaatgcaaaccctggggtgtcatcaatccaaagttaccagggaataggggaaaggcaaatgccgagttgttcctgaacagttcttgcatttcagatacagaaaatacttactaaaagcatctactgcctttgtcagattgttctgggcagactcgttgacttccatgtcctggtcatcagaagactcatcttctcctaggacattttcagaatctggtttccgaatgagaaagaatagaactgtccccacaaggctaatcaccgttagggcaataaacactgttcttcggtcactctctgatatctgagttttcccttgccaggcaaaatatatgtagagatttccaaagaacaagctagactgcagaagtgcccagaaaatcccactgtttctcccaatgctgtgctcatccgaattgattgtcaggcagtttccttgtgctgtccaaagcacagcagcagcaattccaatgaaaacagaggctgtgtagaaggaccacgggaaaggctgtaaaataaaccactggcaaacatagagagttgaggtcctacaatggcaaccactgacggtgtaatcaaatttgaagcagagaacactccatagataatagccatgctggtatatccactgccgtgaaaatctgtcctatttaagctcctgatgacagtttgcgccacatttccacaagtttgaaaggcagtgaacataaacataaaggcaactcctaaaataatgatgttgaaaagctttttagattccggggacattttggctcagctctgccggaggcagcagcccagggcagtcagctctcctcggggcgaagccactgacaatccgcacctcgcccgacacgctgaggcgcgtcttcgagaagtacgggcgcgtcggcgacgtgtacatcccgcgggaccgctacaccaaggagtcccgcggcttcgccttcgttcgctttcacgacaagcgcgacgctgaggacgctatggatgccatggacggggccgtgctggacggccgcgagctgcgggtgcaaatggcgcgctacggccgccccccggactcacaccacagccgccggggaccgccaccccgcaggtacgggggcggtggctacggacgccggagccgcaggtaaacggggctgaggggaccgcgggaggcggggcggggcgcgcgggaggcccgggcgacctcacaaaggtccgcggcgaagcacgtggtgcgggcccggacggggcgggggtgcacgccgcgtctcgcgaccctccggccaccccgcgagcttccgccgtctgc

SEQ ID NO: 15531 - RNA, 2329 nt, Homo sapiens
  source 1..2329: mol_type = other RNA
gctgggattacaggcatgagccactgtgaccagcctattattattttcaagacagggtctcactctgttgcccagcctggagtgcagtggtgtgatcatagctcaccgcagcctcaatctcctgggctgaagtgatccttctgtctcagcctccccaacagctgggagtatagcggtgcaacaccacacccagctttgctatttatttaaatgtcattctccaacacatatggggaatgacatatgcttcccattattacatggcaaaacatactccatatccagaaaaaatatttatatgacatatggcctagtattctaaatcaaggcaggatcttccaacaagagcaggagagagaagaaaacatttacattctataacatgattataagaattgagatagatgaaatgaaaaacaacatctttgaacaattacagttgacagaacagctttcccttattctacttgctttaaataactcatatctgtaaacttgaacaccaactctggctgatttaacagtcttaatcccttgattttccatactgaacatcacccaatatatagtgaagatcaaaggcgacttcttccaccaagctctgtgtccagctgtgtttctgaggtcatacgtgtcccctcacggacaccagatcagatacttcggtagtcagagccgcgggctacaaaggcggcagcttcccattccacagtgaagaaagaaattgttccaaaaaacccaaatatcaccatgaccaggagttgccagtgaaggagaaggtagttgctgtagaaaaatgccacggctgcgcaaatagactgaacaaacttgaagatggcaaatgctggggcgctgtcttcagaatacagaaagcccaagatactaagcagctgggtattaaagcagctgtctccaaggcccaacagaaaactgcagagaatggcaacttctttgctggatttgatgtaagcactgctgtcagttcctttaacaggagcaatcggggcatctccaggcatgttgagaaatattagataaaaagctatgaagtgcaccaggatgcccaacagcacaactggatttctaccaaaacgattgttcttgctcagcaggccgaagaggcttccacctaaaatttctccaatgccgatgaaaatgccagaaagtccaataaggcttttctcttctgctccaaatttatttgtagcaccaatacaggttccatatacaccagagaagaaagttaattccagacctgtataagcagttgtaatactaagaaggagcatctccttggtgacacataacttaaaagacttttctggaaaaatgcaaaccctggggtgtcatcaatccaaagttaccagggaataggggaaaggcaaatgccgagttgttcctgaacagttcttgcatttcagatacagaaaatacttactaaaagcatctactgcctttgtcagattgttctgggcagactcgttgacttccatgtcctggtcatcagaagactcatcttctcctaggacattttcagaatctggtttccgaatgagaaagaatagaactgtccccacaaggctaatcaccgttagggcaataaacactgttcttcggtcactctctgatatctgagttttcccttgccaggcaaaatatatgtagagatttccaaagaacaagctagactgcagaagtgcccagaaaatcccactgtttctcccaatgctgtgctcatccgaattgattgtcaggcagtttccttgtgctgtccaaagcacagcagcagcaattccaatgaaaacagaggctgtgtagaaggaccacgggaaaggctgtaaaataaaccactggcaaacatagagagttgaggtcctacaatggcaaccactgacggtgtaatcaaatttgaagcagagaacactccatagataatagccatgctggtatatccactgccgtgaaaatctgtcctatttaagctcctgatgacagtttgcgccacatttccacaagtttgaaaggcagtgaacataaacataaaggcaactcctaaaataatgatgttgaaaagctttttagattccggggacattttggctcagctctgccggaggcagcagcccagggcagtcagctctcctcggggcgaagccactgacaatcctggagaaagaaatgagatggtgagtggagaaggcagatgcaggagccaggcagccaagctgtcaacttccagttcctggatcggaaccccaggtttagggcgaagttctccccaccggcagttaggatactcctaagaagcgatccgagtacggaagagcac

SEQ ID NO: 15532 - RNA, 1965 nt, Homo sapiens
  source 1..1965: mol_type = other RNA
gctgggattacaggcatgagccactgtgaccagcctattattattttcaagacagggtctcactctgttgcccagcctggagtgcagtggtgtgatcatagctcaccgcagcctcaatctcctgggctgaagtgatccttctgtctcagcctccccaacagctgggagtatagcggtgcaacaccacacccagctttgctatttatttaaatgtcattctccaacacatatggggaatgacatatgcttcccattattacatggcaaaacatactccatatccagaaaaaatatttatatgacatatggcctagtattctaaatcaaggcaggatcttccaacaagagcaggagagagaagaaaacatttacattctataacatgattataagaattgagatagatgaaatgaaaaacaacatctttgaacaattacagttgacagaacagctttcccttattctacttgctttaaataactcatatctgtaaacttgaacaccaactctggctgatttaacagtcttaatcccttgattttccatactgaacatcacccaatatatagtgaagatcaaaggcgacttcttccaccaagctctgtgtccagctgtgtttctgaggtcatacgtgtcccctcacggacaccagatcagatacttcggtagtcagagccgcgggctacaaaggcggcagcttcccattccacagtgaagaaagaaattgttccaaaaaacccaaatatcaccatgaccaggagttgccagtgaaggagaaggtagttgctgtagaaaaatgccacggctgcgcaaatagactgaacaaacttgaagatggcaaatgctggggcgctgtcttcagaatacagaaagcccaagatactaagcagctgggtattaaagcagctgtctccaaggcccaacagaaaactgcagagaatggcaacttctttgctggatttgatgtaagcactgctgtcagttcctttaacaggagcaatcggggcatctccaggcatgttgagaaatattagataaaaagctatgaagtgcaccaggatgcccaacagcacaactggatttctaccaaaacgattgttcttgctcagcaggccgaagaggcttccacctaaaatttctccaatgccgatgaaaatgccagaaagtccaataaggcttttctcttctgctccaaatttatttgtagcaccaatacaggttccatatacaccagagaagaaagttaattccagacctgtataagcagttgtaatactaagaaggagcatctccttggtgacacataacttaaaagactttttaaaagcatctactgcctttgtcagattgttctgggcagactcgttgacttccatgtcctggtcatcagaagactcatcttctcctaggacattttcagaatctggtttccgaatgagaaagaatagaactgtccccacaaggctaatcaccgttagggcaataaacactgttcttcggtcactctcagcagcagcaattccaatgaaaacagaggctgtgtagaaggaccacgggaaaggctggatgaaaacggcaatgtacatgctgtaaaataaaccactggcaaacatagagagttgaggtcctacaatggcaaccactgacggtgtaatcaaatttgaagcagagaacactccatagataatagccatgctggtatatccactgccgtgaaaatctgtcctatttaagctcctgatgacagtttgcgccacatttccacaagtttgaaaggcagtgaacataaacataaaggcaactcctaaaataatgatgttgaaaagctttttagattccggggacattttggctcagctctgccggaggcagcagcccagggcagtcagctctcctcggggcgaagccactgacaatccggcagttaggatactcctaagaagcgatccgagtacggaagagcac

SEQ ID NO: 15533 - RNA, 2217 nt, Homo sapiens
  source 1..2217: mol_type = other RNA
gctgggattacaggcatgagccactgtgaccagcctattattattttcaagacagggtctcactctgttgcccagcctggagtgcagtggtgtgatcatagctcaccgcagcctcaatctcctgggctgaagtgatccttctgtctcagcctccccaacagctgggagtatagcggtgcaacaccacacccagctttgctatttatttaaatgtcattctccaacacatatggggaatgacatatgcttcccattattacatggcaaaacatactccatatccagaaaaaatatttatatgacatatggcctagtattctaaatcaaggcaggatcttccaacaagagcaggagagagaagaaaacatttacattctataacatgattataagaattgagatagatgaaatgaaaaacaacatctttgaacaattacagttgacagaacagctttcccttattctacttgctttaaataactcatatctgtaaacttgaacaccaactctggctgatttaacagtcttaatcccttgattttccatactgaacatcacccaatatatagtgaagatcaaaggcgacttcttccaccaagctctgtgtccagctgtgtttctgaggtcatacgtgtcccctcacggacaccagatcagatacttcggtagtcagagccgcgggctacaaaggcggcagcttcccattccacagtgaagaaagaaattgttccaaaaaacccaaatatcaccatgaccaggagttgccagtgaaggagaaggtagttgctgtagaaaaatgccacggctgcgcaaatagactgaacaaacttgaagatggcaaatgctggggcgctgtcttcagaatacagaaagcccaagatactaagcagctgggtattaaagcagctgtctccaaggcccaacagaaaactgcagagaatggcaacttctttgctggatttgatgtaagcactgctgtcagttcctttaacaggagcaatcggggcatctccaggcatgttgagaaatattagataaaaagctatgaagtgcaccaggatgcccaacagcacaactggatttctaccaaaacgattgttcttgctcagcaggccgaagaggcttccacctaaaatttctccaatgccgatgaaaatgccagaaagtccaataaggcttttctcttctgctccaaatttatttgtagcaccaatacaggttccatatacaccagagaagaaagttaattccagacctgtataagcagttgtaatactaagaaggagcatctccttggtgacacataacttaaaagactttttaaaagcatctactgcctttgtcagattgttctgggcagactcgttgacttccatgtcctggtcatcagaagactcatcttctcctaggacattttcagaatctggtttccgaatgagaaagaatagaactgtccccacaaggctaatcaccgttagggcaataaacactgttcttcggtcactctcagcagcagcaattccaatgaaaacagaggctgtgtagaaggaccacgggaaaggctggatgaaaacggcaatgtacatgctgtaaaataaaccactggcaaacatagagagttgaggtcctacaatggcaaccactgacggtgtaatcaaatttgaagcagagaacactccatagataatagccatgctggtatatccactgccgtgaaaatctgtcctatttaagctcctgatgacagtttgcgccacatttccacaagtttgaaaggcagtgaacataaacataaaggcaactcctaaaataatgatgttgaaaagctttttagattccggggacattttggctcagctctgccggaggcagcagcccagggcagtcagctctcctcggggcgaagccactgacaatcctgaccgcagccgcggcgccggccgctcggcccgctgggaaacgtagtcccgggtggcctggcacgcgcaagcgctccgcggggagtccccaccgccaggacgcagagccgacggagctctcgggctctggcgaaagggggttgggaagcggactccggcgaagagcagtcaggaacggctggacggggccgagagacgacgcagcggagtctgagggggccggggtcacagggagaggcaaatgagggcagaagcactcttcagacggagacggggctgacggctgagcaaaaaaggg

SEQ ID NO: 15534 - RNA, 2178 nt, Homo sapiens
  source 1..2178: mol_type = other RNA
gctgggattacaggcatgagccactgtgaccagcctattattattttcaagacagggtctcactctgttgcccagcctggagtgcagtggtgtgatcatagctcaccgcagcctcaatctcctgggctgaagtgatccttctgtctcagcctccccaacagctgggagtatagcggtgcaacaccacacccagctttgctatttatttaaatgtcattctccaacacatatggggaatgacatatgcttcccattattacatggcaaaacatactccatatccagaaaaaatatttatatgacatatggcctagtattctaaatcaaggcaggatcttccaacaagagcaggagagagaagaaaacatttacattctataacatgattataagaattgagatagatgaaatgaaaaacaacatctttgaacaattacagttgacagaacagctttcccttattctacttgctttaaataactcatatctgtaaacttgaacaccaactctggctgatttaacagtcttaatcccttgattttccatactgaacatcacccaatatatagtgaagatcaaaggcgacttcttccaccaagctctgtgtccagctgtgtttctgaggtcatacgtgtcccctcacggacaccagatcagatacttcggtagtcagagccgcgggctacaaaggcggcagcttcccattccacagtgaagaaagaaattgttccaaaaaacccaaatatcaccatgaccaggagttgccagtgaaggagaaggtagttgctgtagaaaaatgccacggctgcgcaaatagactgaacaaacttgaagatggcaaatgctggggcgctgtcttcagaatacagaaagcccaagatactaagcagctgggtattaaagcagctgtctccaaggcccaacagaaaactgcagagaatggcaacttctttgctggatttgatgtaagcactgctgtcagttcctttaacaggagcaatcggggcatctccaggcatgttgagaaatattagataaaaagctatgaagtgcaccaggatgcccaacagcacaactggatttctaccaaaacgattgttcttgctcagcaggccgaagaggcttccacctaaaatttctccaatgccgatgaaaatgccagaaagtccaataaggcttttctcttctgctccaaatttatttgtagcaccaatacaggttccatatacaccagagaagaaagttaattccagacctgtataagcagttgtaatactaagaaggagcatctccttggtgacacataacttaaaagactttttaaaagcatctactgcctttgtcagattgttctgggcagactcgttgacttccatgtcctggtcatcagaagactcatcttctcctaggacattttcagaatctggtttccgaatgagaaagaatagaactgtccccacaaggctaatcaccgttagggcaataaacactgttcttcggtcactctctagactgcagaagtgcccagaaaatcccactgtttctcccaatgctgtgctcatccgaattgattgtcaggcagtttccttgtgctgtccaaagcacagcagcagcaattccaatgaaaacagaggctgtgtagaaggaccacgggaaaggctggatgaaaacggcaatgtacatgctgtaaaataaaccactggcaaacatagagagttgaggtcctacaatggcaaccactgacggtgtaatcaaatttgaagcagagaacactccatagataatagccatgctggtatatccactgccgtgaaaatctgtcctatttaagctcctgatgacagtttgcgccacatttccacaagtttgaaaggcagtgaacataaacataaaggcaactcctaaaataatgatgttgaaaagctttttagattccggggacattttggctcagctctgccggaggcagcagcccagggcagtcagctctcctcggggcgaagccactgacaatcctggagaaagaaatgagatggtgagtggagaaggcagatgcaggagccaggcagccaagctgtcaacttccagttcctggatcggaaccccaggtttagggcgaagttctccccaccggcagttaggatactcctaagaagcgatccgagtacggaagagcac

SEQ ID NO: 15535 - RNA, 2037 nt, Homo sapiens
  source 1..2037: mol_type = other RNA
gctgggattacaggcatgagccactgtgaccagcctattattattttcaagacagggtctcactctgttgcccagcctggagtgcagtggtgtgatcatagctcaccgcagcctcaatctcctgggctgaagtgatccttctgtctcagcctccccaacagctgggagtatagcggtgcaacaccacacccagctttgctatttatttaaatgtcattctccaacacatatggggaatgacatatgcttcccattattacatggcaaaacatactccatatccagaaaaaatatttatatgacatatggcctagtattctaaatcaaggcaggatcttccaacaagagcaggagagagaagaaaacatttacattctataacatgattataagaattgagatagatgaaatgaaaaacaacatctttgaacaattacagttgacagaacagctttcccttattctacttgctttaaataactcatatctgtaaacttgaacaccaactctggctgatttaacagtcttaatcccttgattttccatactgaacatcacccaatatatagtgaagatcaaaggcgacttcttccaccaagctctgtgtccagctgtgtttctgaggtcatacgtgtcccctcacggacaccagatcagatacttcggtagtcagagccgcgggctacaaaggcggcagcttcccattccacagtgaagaaagaaattgttccaaaaaacccaaatatcaccatgaccaggagttgccagtgaaggagaaggtagttgctgtagaaaaatgccacggctgcgcaaatagactgaacaaacttgaagatggcaaatgctggggcgctgtcttcagaatacagaaagcccaagatactaagcagctgggtattaaagcagctgtctccaaggcccaacagaaaactgcagagaatggcaacttctttgctggatttgatgtaagcactgctgtcagttcctttaacaggagcaatcggggcatctccaggcatgttgagaaatattagataaaaagctatgaagtgcaccaggatgcccaacagcacaactggatttctaccaaaacgattgttcttgctcagcaggccgaagaggcttccacctaaaatttctccaatgccgatgaaaatgccagaaagtccaataaggcttttctcttctgctccaaatttatttgtagcaccaatacaggttccatatacaccagagaagaaagttaattccagacctgtataagcagttgtaatactaagaaggagcatctccttggtgacacataacttaaaagactttttaaaagcatctactgcctttgtcagattgttctgggcagactcgttgacttccatgtcctggtcatcagaagactcatcttctcctaggacattttcagaatctggtttccgaatgagaaagaatagaactgtccccacaaggctaatcaccgttagggcaataaacactgttcttcggtcactctctagactgcagaagtgcccagaaaatcccactgtttctcccaatgctgtgctcatccgaattgattgtcaggcagtttccttgtgctgtccaaagcacagcagcagcaattccaatgaaaacagaggctgtgtagaaggaccacgggaaaggctgtaaaataaaccactggcaaacatagagagttgaggtcctacaatggcaaccactgacggtgtaatcaaatttgaagcagagaacactccatagataatagccatgctggtatatccactgccgtgaaaatctgtcctatttaagctcctgatgacagtttgcgccacatttccacaagtttgaaaggcagtgaacataaacataaaggcaactcctaaaataatgatgttgaaaagctttttagattccggggacattttggctcagctctgccggaggcagcagcccagggcagtcagctctcctcggggcgaagccactgacaatccggcagttaggatactcctaagaagcgatccgagtacggaagagcac

SEQ ID NO: 15536 - RNA, 2161 nt, Homo sapiens
  source 1..2161: mol_type = other RNA
gctgggattacaggcatgagccactgtgaccagcctattattattttcaagacagggtctcactctgttgcccagcctggagtgcagtggtgtgatcatagctcaccgcagcctcaatctcctgggctgaagtgatccttctgtctcagcctccccaacagctgggagtatagcggtgcaacaccacacccagctttgctatttatttaaatgtcattctccaacacatatggggaatgacatatgcttcccattattacatggcaaaacatactccatatccagaaaaaatatttatatgacatatggcctagtattctaaatcaaggcaggatcttccaacaagagcaggagagagaagaaaacatttacattctataacatgattataagaattgagatagatgaaatgaaaaacaacatctttgaacaattacagttgacagaacagctttcccttattctacttgctttaaataactcatatctgtaaacttgaacaccaactctggctgatttaacagtcttaatcccttgattttccatactgaacatcacccaatatatagtgaagatcaaaggcgacttcttccaccaagctctgtgtccagctgtgtttctgaggtcatacgtgtcccctcacggacaccagatcagatacttcggtagtcagagccgcgggctacaaaggcggcagcttcccattccacagtgaagaaagaaattgttccaaaaaacccaaatatcaccatgaccaggagttgccagtgaaggagaaggtagttgctgtagaaaaatgccacggctgcgcaaatagactgaacaaacttgaagatggcaaatgctggggcgctgtcttcagaatacagaaagcccaagatactaagcagctgggtattaaagcagctgtctccaaggcccaacagaaaactgcagagaatggcaacttctttgctggatttgatgtaagcactgctgtcagttcctttaacaggagcaatcggggcatctccaggcatgttgagaaatattagataaaaagctatgaagtgcaccaggatgcccaacagcacaactggatttctaccaaaacgattgttcttgctcagcaggccgaagaggcttccacctaaaatttctccaatgccgatgaaaatgccagaaagtccaataaggcttttctcttctgctccaaatttatttgtagcaccaatacaggttccatatacaccagagaagaaagttaattccagacctgtataagcagttgtaatactaagaaggagcatctccttggtgacacataacttaaaagactttttaaaagcatctactgcctttgtcagattgttctgggcagactcgttgacttccatgtcctggtcatcagaagactcatcttctcctaggacattttcagaatctggtttccgaatgagaaagaatagaactgtccccacaaggctaatcaccgttagggcaataaacactgttcttcggtcactctctgatatctgagttttcccttgccaggcaaaatatatgtagagatttccaaagaacaagctagactgcagaagtgcccagaaaatcccactgtttctcccaatgctgtgctcatccgaattgattgtcaggcagtttccttgtgctgtccaaagcacagcagcagcaattccaatgaaaacagaggctgtgtagaaggaccacgggaaaggctggatgaaaacggcaatgtacatgctaaaatataacaggtcaaggtattacagtcaaacgatacctgtaaaataaaccactggcaaacatagagagttgaggtcctacaatggcaaccactgacggtgtaatcaaatttgaagcagagaacactccatagataatagccatgctggtatatccactgccgtgaaaatctgtcctatttaagctcctgatgacagtttgcgccacatttccacaagtttgaaaggcagtgaacataaacataaaggcaactcctaaaataatgatgttgaaaagctttttagattccggggacattttggctcagctctgccggaggcagcagcccagggcagtcagctctcctcggggcgaagccactgacaatccggcagttaggatactcctaagaagcgatccgagtacggaagagcac

SEQ ID NO: 15537 - RNA, 2277 nt, Homo sapiens
  source 1..2277: mol_type = other RNA
gctgggattacaggcatgagccactgtgaccagcctattattattttcaagacagggtctcactctgttgcccagcctggagtgcagtggtgtgatcatagctcaccgcagcctcaatctcctgggctgaagtgatccttctgtctcagcctccccaacagctgggagtatagcggtgcaacaccacacccagctttgctatttatttaaatgtcattctccaacacatatggggaatgacatatgcttcccattattacatggcaaaacatactccatatccagaaaaaatatttatatgacatatggcctagtattctaaatcaaggcaggatcttccaacaagagcaggagagagaagaaaacatttacattctataacatgattataagaattgagatagatgaaatgaaaaacaacatctttgaacaattacagttgacagaacagctttcccttattctacttgctttaaataactcatatctgtaaacttgaacaccaactctggctgatttaacagtcttaatcccttgattttccatactgaacatcacccaatatatagtgaagatcaaaggcgacttcttccaccaagctctgtgtccagctgtgtttctgaggtcatacgtgtcccctcacggacaccagatcagatacttcggtagtcagagccgcgggctacaaaggcggcagcttcccattccacagtgaagaaagaaattgttccaaaaaacccaaatatcaccatgaccaggagttgccagtgaaggagaaggtagttgctgtagaaaaatgccacggctgcgcaaatagactgaacaaacttgaagatggcaaatgctggggcgctgtcttcagaatacagaaagcccaagatactaagcagctgggtattaaagcagctgtctccaaggcccaacagaaaactgcagagaatggcaacttctttgctggatttgatgtaagcactgctgtcagttcctttaacaggagcaatcggggcatctccaggcatgttgagaaatattagataaaaagctatgaagtgcaccaggatgcccaacagcacaactggatttctaccaaaacgattgttcttgctcagcaggccgaagaggcttccacctaaaatttctccaatgccgatgaaaatgccagaaagtccaataaggcttttctcttctgctccaaatttatttgtagcaccaatacaggttccatatacaccagagaagaaagttaattccagacctgtataagcagttgtaatactaagaaggagcatctccttggtgacacataacttaaaagactttttaaaagcatctactgcctttgtcagattgttctgggcagactcgttgacttccatgtcctggtcatcagaagactcatcttctcctaggacattttcagaatctggtttccgaatgagaaagaatagaactgtccccacaaggctaatcaccgttagggcaataaacactgttcttcggtcactctctgatatctgagttttcccttgccaggcaaaatatatgtagagatttccaaagaacaagctagactgcagaagtgcccagaaaatcccactgtttctcccaatgctgtgctcatccgaattgattgtcaggcagtttccttgtgctgtccaaagcacagcagcagcaattccaatgaaaacagaggctgtgtagaaggaccacgggaaaggctggatgaaaacggcaatgtacatgctaaaatataacaggtcaaggtattacagtcaaacgatacctgtaaaataaaccactggcaaacatagagagttgaggtcctacaatggcaaccactgacggtgtaatcaaatttgaagcagagaacactccatagataatagccatgctggtatatccactgccgtgaaaatctgtcctatttaagctcctgatgacagtttgcgccacatttccacaagtttgaaaggcagtgaacataaacataaaggcaactcctaaaataatgatgttgaaaagctttttagattccggggacattttggctcagctctgccggaggcagcagcccagggcagtcagctctcctcggggcgaagccactgacaatcctggagaaagaaatgagatggtgagtggagaaggcagatgcaggagccaggcagccaagctgtcaacttccagttcctggatcggaaccccaggtttagggcgaagttctccccaccggcagttaggatactcctaagaagcgatccgagtacggaagagcac

SEQ ID NO: 15538 - RNA, 2532 nt, Homo sapiens
  source 1..2532: mol_type = other RNA
gctgggattacaggcatgagccactgtgaccagcctattattattttcaagacagggtctcactctgttgcccagcctggagtgcagtggtgtgatcatagctcaccgcagcctcaatctcctgggctgaagtgatccttctgtctcagcctccccaacagctgggagtatagcggtgcaacaccacacccagctttgctatttatttaaatgtcattctccaacacatatggggaatgacatatgcttcccattattacatggcaaaacatactccatatccagaaaaaatatttatatgacatatggcctagtattctaaatcaaggcaggatcttccaacaagagcaggagagagaagaaaacatttacattctataacatgattataagaattgagatagatgaaatgaaaaacaacatctttgaacaattacagttgacagaacagctttcccttattctacttgctttaaataactcatatctgtaaacttgaacaccaactctggctgatttaacagtcttaatcccttgattttccatactgaacatcacccaatatatagtgaagatcaaaggcgacttcttccaccaagctctgtgtccagctgtgtttctgaggtcatacgtgtcccctcacggacaccagatcagatacttcggtagtcagagccgcgggctacaaaggcggcagcttcccattccacagtgaagaaagaaattgttccaaaaaacccaaatatcaccatgaccaggagttgccagtgaaggagaaggtagttgctgtagaaaaatgccacggctgcgcaaatagactgaacaaacttgaagatggcaaatgctggggcgctgtcttcagaatacagaaagcccaagatactaagcagctgggtattaaagcagctgtctccaaggcccaacagaaaactgcagagaatggcaacttctttgctggatttgatgtaagcactgctgtcagttcctttaacaggagcaatcggggcatctccaggcatgttgagaaatattagataaaaagctatgaagtgcaccaggatgcccaacagcacaactggatttctaccaaaacgattgttcttgctcagcaggccgaagaggcttccacctaaaatttctccaatgccgatgaaaatgccagaaagtccaataaggcttttctcttctgctccaaatttatttgtagcaccaatacaggttccatatacaccagagaagaaagttaattccagacctgtataagcagttgtaatactaagaaggagcatctccttggtgacacataacttaaaagactttttaaaagcatctactgcctttgtcagattgttctgggcagactcgttgacttccatgtcctggtcatcagaagactcatcttctcctaggacattttcagaatctggtttccgaatgagaaagaatagaactgtccccacaaggctaatcaccgttagggcaataaacactgttcttcggtcactctctgatatctgagttttcccttgccaggcaaaatatatgtagagatttccaaagaacaagctagactgcagaagtgcccagaaaatcccactgtttctcccaatgctgtgctcatccgaattgattgtcaggcagtttccttgtgctgtccaaagcacagcagcagcaattccaatgaaaacagaggctgtgtagaaggaccacgggaaaggctggatgaaaacggcaatgtacatgctgtaaaataaaccactggcaaacatagagagttgaggtcctacaatggcaaccactgacggtgtaatcaaatttgaagcagagaacactccatagataatagccatgctggtatatccactgccgtgaaaatctgtcctatttaagctcctgatgacagtttgcgccacatttccacaagtttgaaaggcagtgaacataaacataaaggcaactcctaaaataatgatgttgaaaagctttttagattccggggacattttggctcagctctgccggaggcagcagcccagggcagtcagctctcctcggggcgaagccactgacaatccgcacctcgcccgacacgctgaggcgcgtcttcgagaagtacgggcgcgtcggcgacgtgtacatcccgcgggaccgctacaccaaggagtcccgcggcttcgccttcgttcgctttcacgacaagcgcgacgctgaggacgctatggatgccatggacggggccgtgctggacggccgcgagctgcgggtgcaaatggcgcgctacggccgccccccggactcacaccacagccgccggggaccgccaccccgcaggtacgggggcggtggctacggacgccggagccgcaggtaaacggggctgaggggaccgcgggaggcggggcggggcgcgcgggaggcccgggcgacctcacaaaggtccgcggcgaagcacgtggtgcgggcccggacggggcgggggtgcacgccgcgtctcgcgaccctccggccaccccgcgagcttccgccgtctgc

SEQ ID NO: 15539 - RNA, 2280 nt, Homo sapiens
  source 1..2280: mol_type = other RNA
gctgggattacaggcatgagccactgtgaccagcctattattattttcaagacagggtctcactctgttgcccagcctggagtgcagtggtgtgatcatagctcaccgcagcctcaatctcctgggctgaagtgatccttctgtctcagcctccccaacagctgggagtatagcggtgcaacaccacacccagctttgctatttatttaaatgtcattctccaacacatatggggaatgacatatgcttcccattattacatggcaaaacatactccatatccagaaaaaatatttatatgacatatggcctagtattctaaatcaaggcaggatcttccaacaagagcaggagagagaagaaaacatttacattctataacatgattataagaattgagatagatgaaatgaaaaacaacatctttgaacaattacagttgacagaacagctttcccttattctacttgctttaaataactcatatctgtaaacttgaacaccaactctggctgatttaacagtcttaatcccttgattttccatactgaacatcacccaatatatagtgaagatcaaaggcgacttcttccaccaagctctgtgtccagctgtgtttctgaggtcatacgtgtcccctcacggacaccagatcagatacttcggtagtcagagccgcgggctacaaaggcggcagcttcccattccacagtgaagaaagaaattgttccaaaaaacccaaatatcaccatgaccaggagttgccagtgaaggagaaggtagttgctgtagaaaaatgccacggctgcgcaaatagactgaacaaacttgaagatggcaaatgctggggcgctgtcttcagaatacagaaagcccaagatactaagcagctgggtattaaagcagctgtctccaaggcccaacagaaaactgcagagaatggcaacttctttgctggatttgatgtaagcactgctgtcagttcctttaacaggagcaatcggggcatctccaggcatgttgagaaatattagataaaaagctatgaagtgcaccaggatgcccaacagcacaactggatttctaccaaaacgattgttcttgctcagcaggccgaagaggcttccacctaaaatttctccaatgccgatgaaaatgccagaaagtccaataaggcttttctcttctgctccaaatttatttgtagcaccaatacaggttccatatacaccagagaagaaagttaattccagacctgtataagcagttgtaatactaagaaggagcatctccttggtgacacataacttaaaagactttttaaaagcatctactgcctttgtcagattgttctgggcagactcgttgacttccatgtcctggtcatcagaagactcatcttctcctaggacattttcagaatctggtttccgaatgagaaagaatagaactgtccccacaaggctaatcaccgttagggcaataaacactgttcttcggtcactctctgatatctgagttttcccttgccaggcaaaatatatgtagagatttccaaagaacaagctagactgcagaagtgcccagaaaatcccactgtttctcccaatgctgtgctcatccgaattgattgtcaggcagtttccttgtgctgtccaaagcacagcagcagcaattccaatgaaaacagaggctgtgtagaaggaccacgggaaaggctggatgaaaacggcaatgtacatgctgtaaaataaaccactggcaaacatagagagttgaggtcctacaatggcaaccactgacggtgtaatcaaatttgaagcagagaacactccatagataatagccatgctggtatatccactgccgtgaaaatctgtcctatttaagctcctgatgacagtttgcgccacatttccacaagtttgaaaggcagtgaacataaacataaaggcaactcctaaaataatgatgttgaaaagctttttagattccggggacattttggctcagctctgccggaggcagcagcccagggcagtcagctctcctcggggcgaagccactgacaatccgccaggacgcagagccgacggagctctcgggctctggcgaaagggggttgggaagcggactccggcgaagagcagtcaggaacggctggacggggccgagagacgacgcagcggagtctgagggggccggggtcacagggagaggcaaatgagggcagaagcactcttcagacggagacggggctgacggctgagcaaaaaaggg

SEQ ID NO: 15540 - RNA, 2121 nt, Homo sapiens
  source 1..2121: mol_type = other RNA
gctgggattacaggcatgagccactgtgaccagcctattattattttcaagacagggtctcactctgttgcccagcctggagtgcagtggtgtgatcatagctcaccgcagcctcaatctcctgggctgaagtgatccttctgtctcagcctccccaacagctgggagtatagcggtgcaacaccacacccagctttgctatttatttaaatgtcattctccaacacatatggggaatgacatatgcttcccattattacatggcaaaacatactccatatccagaaaaaatatttatatgacatatggcctagtattctaaatcaaggcaggatcttccaacaagagcaggagagagaagaaaacatttacattctataacatgattataagaattgagatagatgaaatgaaaaacaacatctttgaacaattacagttgacagaacagctttcccttattctacttgctttaaataactcatatctgtaaacttgaacaccaactctggctgatttaacagtcttaatcccttgattttccatactgaacatcacccaatatatagtgaagatcaaaggcgacttcttccaccaagctctgtgtccagctgtgtttctgaggtcatacgtgtcccctcacggacaccagatcagatacttcggtagtcagagccgcgggctacaaaggcggcagcttcccattccacagtgaagaaagaaattgttccaaaaaacccaaatatcaccatgaccaggagttgccagtgaaggagaaggtagttgctgtagaaaaatgccacggctgcgcaaatagactgaacaaacttgaagatggcaaatgctggggcgctgtcttcagaatacagaaagcccaagatactaagcagctgggtattaaagcagctgtctccaaggcccaacagaaaactgcagagaatggcaacttctttgctggatttgatgtaagcactgctgtcagttcctttaacaggagcaatcggggcatctccaggcatgttgagaaatattagataaaaagctatgaagtgcaccaggatgcccaacagcacaactggatttctaccaaaacgattgttcttgctcagcaggccgaagaggcttccacctaaaatttctccaatgccgatgaaaatgccagaaagtccaataaggcttttctcttctgctccaaatttatttgtagcaccaatacaggttccatatacaccagagaagaaagttaattccagacctgtataagcagttgtaatactaagaaggagcatctccttggtgacacataacttaaaagactttttaaaagcatctactgcctttgtcagattgttctgggcagactcgttgacttccatgtcctggtcatcagaagactcatcttctcctaggacattttcagaatctggtttccgaatgagaaagaatagaactgtccccacaaggctaatcaccgttagggcaataaacactgttcttcggtcactctctgatatctgagttttcccttgccaggcaaaatatatgtagagatttccaaagaacaagctagactgcagaagtgcccagaaaatcccactgtttctcccaatgctgtgctcatccgaattgattgtcaggcagtttccttgtgctgtccaaagcacagcagcagcaattccaatgaaaacagaggctgtgtagaaggaccacgggaaaggctggatgaaaacggcaatgtacatgctgtaaaataaaccactggcaaacatagagagttgaggtcctacaatggcaaccactgacggtgtaatcaaatttgaagcagagaacactccatagataatagccatgctggtatatccactgccgtgaaaatctgtcctatttaagctcctgatgacagtttgcgccacatttccacaagtttgaaaggcagtgaacataaacataaaggcaactcctaaaataatgatgttgaaaagctttttagattccggggacattttggctcagctctgccggaggcagcagcccagggcagtcagctctcctcggggcgaagccactgacaatccggcagttaggatactcctaagaagcgatccgagtacggaagagcac

SEQ ID NO: 15541 - RNA, 2196 nt, Homo sapiens
  source 1..2196: mol_type = other RNA
gctgggattacaggcatgagccactgtgaccagcctattattattttcaagacagggtctcactctgttgcccagcctggagtgcagtggtgtgatcatagctcaccgcagcctcaatctcctgggctgaagtgatccttctgtctcagcctccccaacagctgggagtatagcggtgcaacaccacacccagctttgctatttatttaaatgtcattctccaacacatatggggaatgacatatgcttcccattattacatggcaaaacatactccatatccagaaaaaatatttatatgacatatggcctagtattctaaatcaaggcaggatcttccaacaagagcaggagagagaagaaaacatttacattctataacatgattataagaattgagatagatgaaatgaaaaacaacatctttgaacaattacagttgacagaacagctttcccttattctacttgctttaaataactcatatctgtaaacttgaacaccaactctggctgatttaacagtcttaatcccttgattttccatactgaacatcacccaatatatagtgaagatcaaaggcgacttcttccaccaagctctgtgtccagctgtgtttctgaggtcatacgtgtcccctcacggacaccagatcagatacttcggtagtcagagccgcgggctacaaaggcggcagcttcccattccacagtgaagaaagaaattgttccaaaaaacccaaatatcaccatgaccaggagttgccagtgaaggagaaggtagttgctgtagaaaaatgccacggctgcgcaaatagactgaacaaacttgaagatggcaaatgctggggcgctgtcttcagaatacagaaagcccaagatactaagcagctgggtattaaagcagctgtctccaaggcccaacagaaaactgcagagaatggcaacttctttgctggatttgatgtaagcactgctgtcagttcctttaacaggagcaatcggggcatctccaggcatgttgagaaatattagataaaaagctatgaagtgcaccaggatgcccaacagcacaactggatttctaccaaaacgattgttcttgctcagcaggccgaagaggcttccacctaaaatttctccaatgccgatgaaaatgccagaaagtccaataaggcttttctcttctgctccaaatttatttgtagcaccaatacaggttccatatacaccagagaagaaagttaattccagacctgtataagcagttgtaatactaagaaggagcatctccttggtgacacataacttaaaagactttttaaaagcatctactgcctttgtcagattgttctgggcagactcgttgacttccatgtcctggtcatcagaagactcatcttctcctaggacattttcagaatctggtttccgaatgagaaagaatagaactgtccccacaaggctaatcaccgttagggcaataaacactgttcttcggtcactctctgatatctgagttttcccttgccaggcaaaatatatgtagagatttccaaagaacaagctagactgcagaagtgcccagaaaatcccactgtttctcccaatgctgtgctcatccgaattgattgtcaggcagtttccttgtgctgtccaaagcacagcagcagcaattccaatgaaaacagaggctgtgtagaaggaccacgggaaaggctggatgaaaacggcaatgtacatgctgtaaaataaaccactggcaaacatagagagttgaggtcctacaatggcaaccactgacggtgtaatcaaatttgaagcagagaacactccatagataatagccatgctggtatatccactgccgtgaaaatctgtcctatttaagctcctgatgacagtttgcgccacatttccacaagtttgaaaggcagtgaacataaacataaaggcaactcctaaaataatgatgttgaaaagctttttagattccggggacattttggctcagctctgccggaggcagcagcccagggcagtcagctctcctcggggcgaagccactgacaatcctcctcttcctcctgcccaatcgcgatcgtccggcctcccaggcggaaaaagcgtttcgcgggctttccaactgcccgctaattccgctccccctccctccagccgtgactccgcgcttttt

SEQ ID NO: 15542 - RNA, 2527 nt, Homo sapiens
  source 1..2527: mol_type = other RNA
gctgggattacaggcatgagccactgtgaccagcctattattattttcaagacagggtctcactctgttgcccagcctggagtgcagtggtgtgatcatagctcaccgcagcctcaatctcctgggctgaagtgatccttctgtctcagcctccccaacagctgggagtatagcggtgcaacaccacacccagctttgctatttatttaaatgtcattctccaacacatatggggaatgacatatgcttcccattattacatggcaaaacatactccatatccagaaaaaatatttatatgacatatggcctagtattctaaatcaaggcaggatcttccaacaagagcaggagagagaagaaaacatttacattctataacatgattataagaattgagatagatgaaatgaaaaacaacatctttgaacaattacagttgacagaacagctttcccttattctacttgctttaaataactcatatctgtaaacttgaacaccaactctggctgatttaacagtcttaatcccttgattttccatactgaacatcacccaatatatagtgaagatcaaaggcgacttcttccaccaagctctgtgtccagctgtgtttctgaggtcatacgtgtcccctcacggacaccagatcagatacttcggtagtcagagccgcgggctacaaaggcggcagcttcccattccacagtgaagaaagaaattgttccaaaaaacccaaatatcaccatgaccaggagttgccagtgaaggagaaggtagttgctgtagaaaaatgccacggctgcgcaaatagactgaacaaacttgaagatggcaaatgctggggcgctgtcttcagaatacagaaagcccaagatactaagcagctgggtattaaagcagctgtctccaaggcccaacagaaaactgcagagaatggcaacttctttgctggatttgatgtaagcactgctgtcagttcctttaacaggagcaatcggggcatctccaggcatgttgagaaatattagataaaaagctatgaagtgcaccaggatgcccaacagcacaactggatttctaccaaaacgattgttcttgctcagcaggccgaagaggcttccacctaaaatttctccaatgccgatgaaaatgccagaaagtccaataaggcttttctcttctgctccaaatttatttgtagcaccaatacaggttccatatacaccagagaagaaagttaattccagacctgtataagcagttgtaatactaagaaggagcatctccttggtgacacataacttaaaagactttttaaaagcatctactgcctttgtcagattgttctgggcagactcgttgacttccatgtcctggtcatcagaagactcatcttctcctaggacattttcagaatctggtttccgaatgagaaagaatagaactgtccccacaaggctaatcaccgttagggcaataaacactgttcttcggtcactctctgatatctgagttttcccttgccaggcaaaatatatgtagagatttccaaagaacaagctagactgcagaagtgcccagaaaatcccactgtttctcccaatgctgtgctcatccgaattgattgtcaggcagtttccttgtgctgtccaaagcacagcagcagcaattccaatgaaaacagaggctgtgtagaaggaccacgggaaaggctggatgaaaacggcaatgtacatgctgtaaaataaaccactggcaaacatagagagttgaggtcctacaatggcaaccactgacggtgtaatcaaatttgaagcagagaacactccatagataatagccatgctggtatatccactgccgtgaaaatctgtcctatttaagctcctgatgacagtttgcgccacatttccacaagtttgaaaggcagtgaacataaacataaaggcaactcctaaaataatgatgttgaaaagctttttagattccggggacattttggctcagctctgccggaggcagcagcccagggcagtcagctctcctcggggcgaagccactgacaatcctcgcccgacacgctgaggcgcgtcttcgagaagtacgggcgcgtcggcgacgtgtacatcccgcgggaccgctacaccaaggagtcccgcggcttcgccttcgttcgctttcacgacaagcgcgacgctgaggacgctatggatgccatggacggggccgtgctggacggccgcgagctgcgggtgcaaatggcgcgctacggccgccccccggactcacaccacagccgccggggaccgccaccccgcaggtacgggggcggtggctacggacgccggagccgcaggtaaacggggctgaggggaccgcgggaggcggggcggggcgcgcgggaggcccgggcgacctcacaaaggtccgcggcgaagcacgtggtgcgggcccggacggggcgggggtgcacgccgcgtctcgcgaccctccggccaccccgcgagcttccgccgtctgc

SEQ ID NO: 15543 - RNA, 2373 nt, Homo sapiens
  source 1..2373: mol_type = other RNA
gctgggattacaggcatgagccactgtgaccagcctattattattttcaagacagggtctcactctgttgcccagcctggagtgcagtggtgtgatcatagctcaccgcagcctcaatctcctgggctgaagtgatccttctgtctcagcctccccaacagctgggagtatagcggtgcaacaccacacccagctttgctatttatttaaatgtcattctccaacacatatggggaatgacatatgcttcccattattacatggcaaaacatactccatatccagaaaaaatatttatatgacatatggcctagtattctaaatcaaggcaggatcttccaacaagagcaggagagagaagaaaacatttacattctataacatgattataagaattgagatagatgaaatgaaaaacaacatctttgaacaattacagttgacagaacagctttcccttattctacttgctttaaataactcatatctgtaaacttgaacaccaactctggctgatttaacagtcttaatcccttgattttccatactgaacatcacccaatatatagtgaagatcaaaggcgacttcttccaccaagctctgtgtccagctgtgtttctgaggtcatacgtgtcccctcacggacaccagatcagatacttcggtagtcagagccgcgggctacaaaggcggcagcttcccattccacagtgaagaaagaaattgttccaaaaaacccaaatatcaccatgaccaggagttgccagtgaaggagaaggtagttgctgtagaaaaatgccacggctgcgcaaatagactgaacaaacttgaagatggcaaatgctggggcgctgtcttcagaatacagaaagcccaagatactaagcagctgggtattaaagcagctgtctccaaggcccaacagaaaactgcagagaatggcaacttctttgctggatttgatgtaagcactgctgtcagttcctttaacaggagcaatcggggcatctccaggcatgttgagaaatattagataaaaagctatgaagtgcaccaggatgcccaacagcacaactggatttctaccaaaacgattgttcttgctcagcaggccgaagaggcttccacctaaaatttctccaatgccgatgaaaatgccagaaagtccaataaggcttttctcttctgctccaaatttatttgtagcaccaatacaggttccatatacaccagagaagaaagttaattccagacctgtataagcagttgtaatactaagaaggagcatctccttggtgacacataacttaaaagactttttaaaagcatctactgcctttgtcagattgttctgggcagactcgttgacttccatgtcctggtcatcagaagactcatcttctcctaggacattttcagaatctggtttccgaatgagaaagaatagaactgtccccacaaggctaatcaccgttagggcaataaacactgttcttcggtcactctctgatatctgagttttcccttgccaggcaaaatatatgtagagatttccaaagaacaagctagactgcagaagtgcccagaaaatcccactgtttctcccaatgctgtgctcatccgaattgattgtcaggcagtttccttgtgctgtccaaagcacagcagcagcaattccaatgaaaacagaggctgtgtagaaggaccacgggaaaggctggatgaaaacggcaatgtacatgctgtaaaataaaccactggcaaacatagagagttgaggtcctacaatggcaaccactgacggtgtaatcaaatttgaagcagagaacactccatagataatagccatgctggtatatccactgccgtgaaaatctgtcctatttaagctcctgatgacagtttgcgccacatttccacaagtttgaaaggcagtgaacataaacataaaggcaactcctaaaataatgatgttgaaaagctttttagattccggggacattttggctcagctctgccggaggcagcagcccagggcagtcagctctcctcggggcgaagccactgacaatcctgaccgcagccgcggcgccggccgctcggcccgctgggaaacgtagtcccgggtggcctggcacgcgcaagcgctccgcggggagtccccaccgccaggacgcagagccgacggagctctcgggctctggcgaaagggggttgggaagcggactccggcgaagagcagtcaggaacggctggacggggccgagagacgacgcagcggagtctgagggggccggggtcacagggagaggcaaatgagggcagaagcactcttcagacggagacggggctgacggctgagcaaaaaaggg

SEQ ID NO: 15544 - RNA, 2237 nt, Homo sapiens
  source 1..2237: mol_type = other RNA
gctgggattacaggcatgagccactgtgaccagcctattattattttcaagacagggtctcactctgttgcccagcctggagtgcagtggtgtgatcatagctcaccgcagcctcaatctcctgggctgaagtgatccttctgtctcagcctccccaacagctgggagtatagcggtgcaacaccacacccagctttgctatttatttaaatgtcattctccaacacatatggggaatgacatatgcttcccattattacatggcaaaacatactccatatccagaaaaaatatttatatgacatatggcctagtattctaaatcaaggcaggatcttccaacaagagcaggagagagaagaaaacatttacattctataacatgattataagaattgagatagatgaaatgaaaaacaacatctttgaacaattacagttgacagaacagctttcccttattctacttgctttaaataactcatatctgtaaacttgaacaccaactctggctgatttaacagtcttaatcccttgattttccatactgaacatcacccaatatatagtgaagatcaaaggcgacttcttccaccaagctctgtgtccagctgtgtttctgaggtcatacgtgtcccctcacggacaccagatcagatacttcggtagtcagagccgcgggctacaaaggcggcagcttcccattccacagtgaagaaagaaattgttccaaaaaacccaaatatcaccatgaccaggagttgccagtgaaggagaaggtagttgctgtagaaaaatgccacggctgcgcaaatagactgaacaaacttgaagatggcaaatgctggggcgctgtcttcagaatacagaaagcccaagatactaagcagctgggtattaaagcagctgtctccaaggcccaacagaaaactgcagagaatggcaacttctttgctggatttgatgtaagcactgctgtcagttcctttaacaggagcaatcggggcatctccaggcatgttgagaaatattagataaaaagctatgaagtgcaccaggatgcccaacagcacaactggatttctaccaaaacgattgttcttgctcagcaggccgaagaggcttccacctaaaatttctccaatgccgatgaaaatgccagaaagtccaataaggcttttctcttctgctccaaatttatttgtagcaccaatacaggttccatatacaccagagaagaaagttaattccagacctgtataagcagttgtaatactaagaaggagcatctccttggtgacacataacttaaaagactttttaaaagcatctactgcctttgtcagattgttctgggcagactcgttgacttccatgtcctggtcatcagaagactcatcttctcctaggacattttcagaatctggtttccgaatgagaaagaatagaactgtccccacaaggctaatcaccgttagggcaataaacactgttcttcggtcactctctgatatctgagttttcccttgccaggcaaaatatatgtagagatttccaaagaacaagctagactgcagaagtgcccagaaaatcccactgtttctcccaatgctgtgctcatccgaattgattgtcaggcagtttccttgtgctgtccaaagcacagcagcagcaattccaatgaaaacagaggctgtgtagaaggaccacgggaaaggctggatgaaaacggcaatgtacatgctgtaaaataaaccactggcaaacatagagagttgaggtcctacaatggcaaccactgacggtgtaatcaaatttgaagcagagaacactccatagataatagccatgctggtatatccactgccgtgaaaatctgtcctatttaagctcctgatgacagtttgcgccacatttccacaagtttgaaaggcagtgaacataaacataaaggcaactcctaaaataatgatgttgaaaagctttttagattccggggacattttggctcagctctgccggaggcagcagcccagggcagtcagctctcctcggggcgaagccactgacaatcctggagaaagaaatgagatggtgagtggagaaggcagatgcaggagccaggcagccaagctgtcaacttccagttcctggatcggaaccccaggtttagggcgaagttctccccaccggcagttaggatactcctaagaagcgatccgagtacggaagagcac

SEQ ID NO: 15545 - RNA, 2395 nt, Homo sapiens
  source 1..2395: mol_type = other RNA
gctgggattacaggcatgagccactgtgaccagcctattattattttcaagacagggtctcactctgttgcccagcctggagtgcagtggtgtgatcatagctcaccgcagcctcaatctcctgggctgaagtgatccttctgtctcagcctccccaacagctgggagtatagcggtgcaacaccacacccagctttgctatttatttaaatgtcattctccaacacatatggggaatgacatatgcttcccattattacatggcaaaacatactccatatccagaaaaaatatttatatgacatatggcctagtattctaaatcaaggcaggatcttccaacaagagcaggagagagaagaaaacatttacattctataacatgattataagaattgagatagatgaaatgaaaaacaacatctttgaacaattacagttgacagaacagctttcccttattctacttgctttaaataactcatatctgtaaacttgaacaccaactctggctgatttaacagtcttaatcccttgattttccatactgaacatcacccaatatatagtgaagatcaaaggcgacttcttccaccaagctctgtgtccagctgtgtttctgaggtcatacgtgtcccctcacggacaccagatcagatacttcggtagtcagagccgcgggctacaaaggcggcagcttcccattccacagtgaagaaagaaattgttccaaaaaacccaaatatcaccatgaccaggagttgccagtgaaggagaaggtagttgctgtagaaaaatgccacggctgcgcaaatagactgaacaaacttgaagatggcaaatgctggggcgctgtcttcagaatacagaaagcccaagatactaagcagctgggtattaaagcagctgtctccaaggcccaacagaaaactgcagagaatggcaacttctttgctggatttgatgtaagcactgctgtcagttcctttaacaggagcaatcggggcatctccaggcatgttgagaaatattagataaaaagctatgaagtgcaccaggatgcccaacagcacaactggatttctaccaaaacgattgttcttgctcagcaggccgaagaggcttccacctaaaatttctccaatgccgatgaaaatgccagaaagtccaataaggcttttctcttctgctccaaatttatttgtagcaccaatacaggttccatatacaccagagaagaaagttaattccagacctgtataagcagttgtaatactaagaaggagcatctccttggtgacacataacttaaaagactttttaaaagcatctactgcctttgtcagattgttctgggcagactcgttgacttccatgtcctggtcatcagaagactcatcttctcctaggacattttcagaatctggtttccgaatgagaaagaatagaactgtccccacaaggctaatcaccgttagggcaataaacactgttcttcggtcactctctgatatctgagttttcccttgccaggcaaaatatatgtagagatttccaaagaacaagctagactgcagaagtgcccagaaaatcccactgtttctcccaatgctgtgctcatccgaattgattgtcaggcagtttccttgtgctgtccaaagcacagcagcagcaattccaatgaaaacagaggctgtgtagaaggaccacgggaaaggctggatgaaaacggcaatgtacatgctgtaaaataaaccactggcaaacatagagagttgaggtcctacaatggcaaccactgacggtgtaatcaaatttgaagcagagaacactccatagataatagccatgctggtatatccactgccgtgaaaatctgtcctatttaagctcctgatgacagtttgcgccacatttccacaagtttgaaaggcagtgaacataaacataaaggcaactcctaaaataatgatgttgaaaagctttttagattccggggacattttggctcagctctgccggaggcagcagcccagggcagtcagctctcctcggggcgaagccactgacaatctgcggccaggcgaccgggtcacctgaccgcagccgcggcgccggccgctcggcccgctgggaaacgtagtcccgggtggcctggcacgcgcaagcgctccgcggggagtccccaccgccaggacgcagagccgacggagctctcgggctctggcgaaagggggttgggaagcggactccggcgaagagcagtcaggaacggctggacggggccgagagacgacgcagcggagtctgagggggccggggtcacagggagaggcaaatgagggcagaagcactcttcagacggagacggggctgacggctgagcaaaaaaggg

SEQ ID NO: 15546 - RNA, 65 nt, Homo sapiens
  source 1..65: mol_type = other RNA
gctgggattacaggcatgagccactgtgaccagcctccgtgtaaatctatacaatctattcctca

SEQ ID NO: 15547 - RNA, 78 nt, Homo sapiens
  source 1..78: mol_type = other RNA
gctgggattacaggcatgagccactgtgaccagcctccgtgtaaatctatacaatctattcctcagctcctttccaga

SEQ ID NO: 15548 - RNA, 3540 nt, Homo sapiens
  source 1..3540: mol_type = other RNA
gctgggattacaggcatgagccactgtgccaggccaacattgtttttaatatatgacttgtaaggcaagttggggggcattaattccttattaagatgtactgagttgaataaaagcccctccaaccatcaaccccccaaaatatatgtccaagtactaagctccagaatttgtgaatgcaaactaatttggataaagagtatttgcatgtaattaaggaaagattcttgagattagatcactataaattacccaggtggcctttaaatccaatgaccagtgtccttctaagagacagaagaggagacacagacacagaggaaaaggtcacgtggagatggaggcagagaatgtagtgatgtggccacaagcccagggacacctggagccaccaggagctggaagaggcaggaaggatcctctcctagaacctccagggggagcgcacccctgcccacaccttgatctcagattcctggtctccaatactggaaaagagtaaacatctgttactttacaccatccaagtttttgttatttgctacggcatccataggaattaaaaacctataggtatgaattttatgttgctgtcaaaaggcttcttctaggataagtagatatttcacctagatagttgtagctttttctcctcttcattgggatcggaactcagttggtgtcctccatcctcctatctcaatattgattttacttactctttaatcctaacaatgagcctttttatattgcttaattaaatatcaatgtctttctggtcaacatgagaccaaaaacctttttaccttgggcctgagaaagagcagtatttctcctcctcctcttcctcttcttcctcctccttccttcttctccctctttttagagatggggtctctctctgttgcccaggctagagtgcagtggcataatcctagctcactgcagcctcaaactcctgggctcaagtgatcttccagcctcagcctgctgagtaactgggaccacacatgtgcaccactgtgccctatttttttgtttttttaacttatttatagaaatgaggtctcactatgttgcccaggctggtctcatacttctggcctcaagtgttcctcctctttggcctcccaaagcactgggattacaggtgtgagccaccatgctttggcatggtggggtatgcagtaggagagcaggggtggtggcagtgtctccatatgtactctcactaaaactggtgtgggcagatactggatgcctacttatttaggggcatctaaattcctgtgctaaattagaaaatagaggcagctcttgaaaggagtgatggcatgaaggagagatgcttggaccaaccaccacacaacccttataaataattgataaccttggttttgatgccacgtcctcttcgacagttgttggttgaaatgacacatgattccaggtgagcttttccagataaattgccctggaacttcagactttgtcgggtgaatcgatgtggaatttcagaatgggctggaatgtctaagatgggcatgtccaatattcagctcagtgtggggaaactggtggtggccagggctggttgcaagctgagttgtaggggtgacagttcacctgtaaatggagtgcataggcagcagtgcttctcccccaaggctggggcgatggaatcagttagactactgagggcatctggaagggcatctgtgtcagggttagtcctcagggtatggtggccaatgggtttcttttggttgactgttgacaatgcgtttgttgaatggcagcctgcactaggtgacgctgaagccacagaagacacattgtttatttccagggtctcctgagaacacagaccagaattactgaggtaatcttggcacattttcttaaccattttatgcgactttcaaattccttatatgtagctgggaaaaaaggctttgctagatgatctttttcaactggtggtacgtgactgtagtcccagctactcgggaggttgaggcaggagaatcacttgaacctgggaggtggaggttgtagtgaactcagactgctccactgtactccagcctgggcgacagagtgagaccaggccaccgcgtgctgactctctcaccaagcaggagcgggcccctccctcacgcggagccgctggcacggacagccccgggaaggtcaggctgagcgtcctttcctctgtgcacccacggagggtgctcccattggctttctcagatagcaccatctcagggtccagctggccatggcctggattaagtttaaaatgctgggccagtccccacttccctatatatgactttttacaagtctgacacttgaagcttttgggcctcagggagcagcttgataagtcaaagagcgcctgcctctccctctgatgttcttccacactgagttctgaatcatcatcagaatctggcagatgaccgtcggccaaatcatccctttttatgaactcagctttagctgtatacttggcaggtcgagatacctgtctcaacgtgtcttcacttttaacgatggttttagtttctcagtatgttttgtatgcaagttggaaataaataaacgtcctgaactggatgaaacatgttacagtcggcgaactggaggccaacgaaggggtcaacatggtgccctgtccatttggagccttgggagctgggactctctttgcagggaccacctagagggctggcagtggtctctgtacaaacccctgagcaggaggctgatgtaggaaacatgactgtggctcggttctcacgaggggctgtaccctgagcagctgggggctggtgacgtggagtcccaccaggcgggaattcccccggggcggctggctctgtcttgcagattggggctggactgtggccagtagggacgttggccgttcctgaccttttgtttctccagacgttaccttgacacaaatggcttctagttgctttcccacggtgaccagcgtgtcgaagtcttgaaggcggttggcaggcggctccggcgaccgcgactcggggctggggcagagctcgggcgcccagtccggggtctcctctgccacggccgcctgggccagcccgggcgccttcatggggacgcactcaggtccggggcgccgggccgggccggagcgctcggggagccgggcttccgcggatgcagcctcggagggcggcgcggcggcatcaacggaggctccccatgcgcgccatgcggcttgtggaggccatcctgcccacccggcccggagcccgcaagacgccaatgcgccttccggtgcgcgcgcggccgggcgcggctgacggagcggcggggacaatggctggccgtcgctcacggcacaagcagcaacggccccaggtagcagcagccgccggcctcgtggggcgggcacggagcgccgggaggcggcggggaaggcgggggccgcggcccgggcttgtagagccaggcgggggccctgcgcattcccagtctcgcgcccgcggcctcctgcag

SEQ ID NO: 15549 - RNA, 1660 nt, Homo sapiens
  source 1..1660: mol_type = other RNA
gctgggattacaggcatgagccactgtgccaggccaacattgtttttaatatatgacttgtaaggcaagttggggggcattaattccttattaagatgtactgagttgaataaaagcccctccaaccatcaaccccccaaaatatatgtccaagtactaagctccagaatttgtgaatgcaaactaatttggataaagagtatttgcatgtaattaaggaaagattcttgagattagatcactataaattacccaggtggcctttaaatccaatgaccagtgtccttctaagagacagaagaggagacacagacacagaggaaaaggtcacgtggagatggaggcagagaatgtagtgatgtggccacaagcccagggacacctggagccaccaggagctggaagaggcaggaaggatcctctcctagaacctccagggggagcgcacccctgcccacaccttgatctcagattcctggtctccaatactggaaaagagtaaacatctgttactttacgccatccaagtttttgttatttgctacggcatccataggaattaaaaacctataggtatgaattttatgttgctgtcaaaaggcttcttctaggataagtagatatttcacctagatagttgtagctttttctcctcttcattgggatcggaactcagttggtgtcctccatcctcctatctcaatattgattttacttactctttaatcctaacaatgagcctttttatattgcttaattaaatatcaatgtctttctggtcaacatgagaccaaaaacctttttaccttgggcctgagaaagagcagtatttctcctcctcctcttcctcttcttcctcctccttccttcttctccctctttttagagatggggtctctctctgttgcccaggctagagtgcagtggcataatcctagctcactgcagcctcaaactcctgggctcaagtgatcttccagcctcagcctgctgagtaactgggaccacacatgtgcaccactatgccctatttttttgtttttttaacttatttatagaaatgaggtctcactatgttgcccaggctggtctcatacttctggcctcaagtgttcctcctctttggcctcccaaagcactgggattacaggtgtgagccaccatgctttggcatggtggggtatgcagtaggagagcaggggtggtggtagtgtctccatatgtactctcactaaaactggtgtgggcagatactggatgcctacttatttaggggcatctaaattcctgtgctaaattagaaaatagaggcagctcttgaaaggagtgatggcatgaaggagagatgcttggaccaaccaccacacaacccttataaataattgataaccttggttttgatgccacgtcctcttcgacagttgttggttgaaatgacacatgattccaggtgagcttttccagataaattgccctggaacttcagactttgtcgggtgaatcgatgtggaatttcagaatgggctggaatgtctaagatgggcatgtccaatattcagctcagtgtggggaaactggtggtggccagggctggttgcaagctgagttgtaggggtgacagttcacctgtaaatggagtgcataggcagcagtgcttctc

SEQ ID NO: 15550 - RNA, 758 nt, Homo sapiens
  source 1..758: mol_type = other RNA
gctgggattacaggcatgagccactgtgccaggccaacattgtttttaatatatgacttgtaaggcaagttggggggcattaattccttattaagatgtactgagttgaataaaagcccctccaaccatcaaccccccaaaatatatgtccaagtactaagctccagaatttgtgaatgcaaactaatttggataaagagtatttgcatgtaattaaggaaagattcttgagattagatcactataaattacccaggtggcctttaaatccaatgaccagtgtccttctaagagacagaagaggagacacagacacagaggaaaaggtcacgtggagatggaggcagagaatgtagtgatgtggccacaagcccagggacacctggagccaccaggagctggaagaggcaggaaggatcctctcctagaacctccagggggagcgcacccctgcccacaccttgatctcagattcctggtctccaatacttggttttgatgccacgtcctcttcgacagttgttggttgaaatgacacatgattccaggtgagcttttccagataaattgccctggaacttcagactttgtcgggtgaatcgatgtggaatttcagaatgggctggaatgtctaagatgggcatgtccaatattcagctcagtgtggggaaactggtggtggccagggctggttgcaagctgagttgtaggggtgacagttcacctgtaaatggagtgcataggcagcagtgcttctc

SEQ ID NO: 15551 - RNA, 3120 nt, Homo sapiens
  source 1..3120: mol_type = other RNA
gctgggattacaggcatgagccactgtgccaggccccttttctttccttaaatggggatctcccactgccttgggaacgagataatcaaaccaattagagctatatgtaaaatgaaagtaaaataggcctgaagggctggcccacaaggaccccataagagcccagattccttaacttccactttcatgtcagagcagccccactgcatacctcttttgtgctgtgtcccagataaaggagtacatcatgtcaccgagttctaagtaagtggggtgcactgaaactttcagtagaagcaagatgcaaacacatacaaacatgtatgatgttatttattttctcactggcactggcctactgcacttaaacatttccatcagactcaaaaaataattttatttcagaaaaaatattttacctatttagcttttgtttatactgttttattattaataggtttttttttctttttttaagagataggatcttgctgtgttgcccaggctgatctccaattcctggcttcaagcaatcctcctgtctcagcctcctgtgcagctgggactataggtatatgccactgctcccagcttgacttaatggaatgtgtttttattcacccattggaaaagcctttgctacatattaatacaaacttctcattaataaaccctccttttttttttttttgagacggagtctcgctctgtcgctcaggtacgatctcgactcactgtaacctcctccgcctggggtcaagcaattctcccgtctcagcctcctgagtacctgggattacaggtgcacgccaccatgcccagccactaataaatccttctttaagtaagaaaataatataacatgagcataactttgcatgaattttaatgtcctggaggcttgttgctttgtataaagtgcaggtcagtaaaaattaaaatgaggtaatgtggtataatacgattaacccagtaagggtacaataaaggatggctattattattattatattgttattattattttgagacagagttttgctcagtcacccaggttacagtgcaatggcacgatctcggctcactgcaacctccacctctgggttcaagcgattcttccgcttcagcctcccaagtagctgggattacaggcacctgccatcatgcccggctaattttttgtatttttagtagagacggggtttcatcatgttggccaggctggtcttgaactcctgacctcaggtgatccacccaccttggcctccaaaagtgctgggattacaggtgtgagccaccgcgccaggccaaggatggctattattttcacatgaattcaactgaaatcacgatagggcaacaccaataacaatgtttcctatatagcttaaaaactgttctttgtcatcccctcatctacccaatagggaattagaactagcctgttaggttgcttgacaggaccactgaatgctgggaatcaaccatactctattctctcatttaacagatggggaagcagaggtccagggaatttgggaaacttgtccacaaagggacaactactttgtggctgaactatgtctaggaccagggctctctttatcaacatgagtatctccttcctttatctgccccttcatgtttacaaggcacctcctcagctccatgattttgtttgttacgctacatcactcagctcatgaaaacggctttttttcctcttttcttgtctttggaagattttttgcattcttgtagcagctgattccatactaacctttaaattgaaaaaatatatatacacacagacacgtatgtgaatatgtgggagaaacagcactaggtctccctggacaacccagtgcaggccacaccttggcagtcacagagcacaaataagaaatgatcttcccgtgtgagttgctttcgacacttcaatgctaaagagctcagaagtgcttacactttgaaagaagcctgaaaacatttgtaggctaccctttaatgtgtctcatttggagatagaacagtgagcaggttgaccagctgctcttcatgtacttcttgcagtaaatccttcaaagaatgaagagtgaagacaattcattttccctcctggaatttttccttcttattattttgcttttttaaaggttgttatattcaggtataggcataagacattataaaagataaggggtatcatgtgagggaggaaatccgacaatccaaaaaatcttccatagaaattaaaaatcagaacttgggggcaaggtaggaggcaacacattctttctacagagctgtgacacatagcccaactgtcctcaaaagcaggaataaaaaaaataaacaacaacaacaacaaaaaacagacctcagctgcataatgaagctggggtcttggcctgatagcttttaatgtccttaaaacggggctgggcatcaagcatcttttccggaataggccaaggaagacaagtccagtttggtttttaaggctttagtgagctctgcggccagcagctcatggagggacacgccgtcgtgggagtacacccagtttttcccagtccagtcataacgcttaggtccactacatacctggatggagaagatagccagatttgcttgtttggcgtctgcttgttgatcacataggttcctagatctccacccagtttgacagttaagacaccactcccaaaggagacatcatagtcctcaaacgtgtatggcttgtctgcaaggtcttcaaaaaactctgctaaagagtccagcgtttcctctgctagtctttcataggtggtctcatctagagagcctgggtggcccaaagttccagatttcctcaaattcatcaaatagacactctgctttttgacattccaaatctggttgaggccacgttggttcgaacttgcgcggcggggcgtgcaggtcgcatcgatgtcggtgcgcaggccacggcggccgcagagtggggccaactctgccggccgcgggacccgggtgagggtctgggcctgggctgggctgggtgacgccaggaggccggctactgcgcggcgcccgagagtccacatgctgctccgggtctgccgcccgctccgccct

SEQ ID NO: 15552 - RNA, 3112 nt, Homo sapiens
  source 1..3112: mol_type = other RNA
gctgggattacaggcatgagccactgtgccaggccccttttctttccttaaatggggatctcccactgccttgggaacgagataatcaaaccaattagagctatatgtaaaatgaaagtaaaataggcctgaagggctggcccacaaggaccccataagagcccagattccttaacttccactttcatgtcagagcagccccactgcatacctcttttgtgctgtgtcccagataaaggagtacatcatgtcaccgagttctaagtaagtggggtgcactgaaactttcagtagaagcaagatgcaaacacatacaaacatgtatgatgttatttattttctcactggcactggcctactgcacttaaacatttccatcagactcaaaaaataattttatttcagaaaaaatattttacctatttagcttttgtttatactgttttattattaataggtttttttttctttttttaagagataggatcttgctgtgttgcccaggctgatctccaattcctggcttcaagcaatcctcctgtctcagcctcctgtgcagctgggactataggtatatgccactgctcccagcttgacttaatggaatgtgtttttattcacccattggaaaagcctttgctacatattaatacaaacttctcattaataaaccctccttttttttttttttgagacggagtctcgctctgtcgctcaggtacgatctcgactcactgtaacctcctccgcctggggtcaagcaattctcccgtctcagcctcctgagtacctgggattacaggtgcacgccaccatgcccagccactaataaatccttctttaagtaagaaaataatataacatgagcataactttgcatgaattttaatgtcctggaggcttgttgctttgtataaagtgcaggtcagtaaaaattaaaatgaggtaatgtggtataatacgattaacccagtaagggtacaataaaggatggctattattattattatattgttattattattttgagacagagttttgctcagtcacccaggttacagtgcaatggcacgatctcggctcactgcaacctccacctctgggttcaagcgattcttccgcttcagcctcccaagtagctgggattacaggcacctgccatcatgcccggctaattttttgtatttttagtagagacggggtttcatcatgttggccaggctggtcttgaactcctgacctcaggtgatccacccaccttggcctccaaaagtgctgggattacaggtgtgagccaccgcgccaggccaaggatggctattattttcacatgaattcaactgaaatcacgatagggcaacaccaataacaatgtttcctatatagcttaaaaactgttctttgtcatcccctcatctacccaatagggaattagaactagcctgttaggttgcttgacaggaccactgaatgctgggaatcaaccatactctattctctcatttaacagatggggaagcagaggtccagggaatttgggaaacttgtccacaaagggacaactactttgtggctgaactatgtctaggaccagggctctctttatcaacatgagtatctccttcctttatctgccccttcatgtttacaaggcacctcctcagctccatgattttgtttgttacgctacatcactcagctcatgaaaacggctttttttcctcttttcttgtctttggaagattttttgcattcttgtagcagctgattccatactaacctttaaattgaaaaaatatatatacacacagacacgtatgtgaatatgtgggagaaacagcactaggtctccctggacaacccagtgcaggccacaccttggcagtcacagagcacaaataagaaatgatcttcccgtgtgagttgctttcgacacttcaatgctaaagagctcagaagtgcttacactttgaaagaagcctgaaaacatttgtaggctaccctttaatgtgtctcatttggagatagaacagtgagcaggttgaccagctgctcttcatgtacttcttgcagtaaatccttcaaagaatgaagagtgaagacaattcattttccctcctggaatttttccttcttattattttgcttttttaaaggttgttatattcaggtataggcataagacattataaaagataaggggtatcatgtgagggaggaaatccgacaatccaaaaaatcttccatagaaattaaaaatcagaacttgggggcaaggtaggaggcaacacattctttctacagagctgtgacacatagcccaactgtcctcaaaagcaggaataaaaaaaataaacaacaacaacaacaaaaaacagacctcagctgcataatgaagctggggtcttggcctgatagcttttaatgtccttaaaacggggctgggcatcaagcatcttttccggaataggccaaggaagacaagtccagtttggtttttaaggctttagtgagctctgcggccagcagctcatggagggacacgccgtcgtgggagtacacccagtttttcccagtccagtcataacgcttaggtccactggatggagaagatagccagatttgcttgtttggcgtctgcttgttgatcacataggttcctagatctccacccagtttgacagttaagacaccactcccaaaggagacatcatagtcctcaaacgtgtatggcttgtctgcaaggtcttcaaaaaactctgctaaagagtccagcgtttcctctgctagtctttcataggtggtctcatctagagagcctgggtggcccaaagttccagatttcctcaaattcatcaaatagacactctgctttttgacattccaaatctggttgaggccacgttggttcgaacttgcgcggcggggcgtgcaggtcgcatcgatgtcggtgcgcaggccacggcggccgcagagtggggccaactctgccggccgcgggacccgggtgagggtctgggcctgggctgggctgggtgacgccaggaggccggctactgcgcggcgcccgagagtccacatgctgctccgggtctgccgcccgctccgccct

SEQ ID NO: 15553 - RNA, 3444 nt, Homo sapiens
  source 1..3444: mol_type = other RNA
gctgggattacaggcatgagccactgtgccaggcctgttcttagggaaagctttttaggtttattaatgaaaatcctaatgttactaattgagacatcagttaacacccaacttagtgattcccatccaaccataattatgtatttttcaagaaaatacataatttactaacacattttccttaccatagccattttcaaaagaaggtagggtactaacactttccagtttagatggccaaagcccggtcagtctctataattaaacaattattttaaaccctagttatgctaaaaccaagctattcttatcacaagtcccattctgctaaccacaaaatttagagaatttgtacctggaagataccaccacgtgtcaattacaatatacgtattccttggtcaattctgatatcacaggaccggaaaaaatagctgcttggtgtctagattgtttgggtattaaaaccactgcacatggataagctatttgttcagtcggagagaaagggcatagagtgacagagcaacaaaaagacacacagagaatgtatttcttgtgaaagaaaagaatgaaatgaaatgaaatgtagaaaccctaatggccttttgctttggaaaattaactccacaagccactaaaaatactatcaattagatcagaaaagacattcggtatgtatgtgttcctcaagcattttagaaaggggatatgctataacttccctgttggttccagattcaacacagcacaaagcaagaaaacttttatttactacactcacaagtatgattaagtgttcctgtttactctggtaggttaaaatatcaaatattagttcccacagaagaacttttttttaaacatctaatcctattcgaaggataaaaggggaaaaactcattaaatgttgaacactgccactttaagtaccatttttgtcttcgggtgaatgtacataagactaaatcatgatccaacaatagttttctatttggtttcactagtatcactcaaagaacttgacacaggctaatgctttaacactttcttatctgagacaaatttaactctaagaacatatgactcaacaatgtacaaagatttaagaatttgccaatctgtcaatcattttaaagagtccatataatatacacatagcaatataatattcataaccagaaactgcactaagtaaacacatcatttagtttaagctctacctgaaaacatgctgttttattaaaacaaaacccaaagacttaaatctcaagttatatggttttacaattaagtcttactgaagcagcacagatttcctttcttacaaacaagttaatatgcaggaagaacccacaaagtgcacaccaacaatgtgacaaattgtaatatgtgaaatacaaataaatcctgaagttaatctgaagaatgtcaaggagttaccagagaggttatgtagtgcccttgatttttattttacctacaagtctacaaattctaaaatttactcaattgatttaacttttttaataaacagcaccagtcttgcccattgatacaattaaaatttgaccttctcagttcttagttcacaagtttattatgaaaaacactgcagtgctcttgtgcagtcacatcgtcttacaggaaggggaaaaaacagttctgttcaaaacaactcaccaggttctgacaataacaaagaacaacatggggctgagatttgagtagggaataaactgagtgcagacaaatcatataattaaattaaacggtatccctgaaaataaaaagaacaatttcaaaactcacaagtagaagggaggccttggtaattatttttaaaaatgttcattaagctccaatgattgtttgctgctatccttatctacagtcatgctgagtaaagctatagctaaatggaagttaaattgtattcacgaggtgttaatgtttacatcttattatctgcagtctctcagagaaagcaaaagtaactacaaatagcgctatgccagaaactggtttcttgaccaacaatgtcgcttcagcatgcaatgaactggttcattctaaagtggtcacggctgttgatgacaagaggctttgtatttttatatggcacatcttttggtccatgtgaaaacaagttttttgaatgttaactattttctgacactttggagttactgttgctcttcccatttccattaggtcgatatatggttcatggcaatactgtacaagtttaaaatttcattacaggaagtagtctggggtacgacgagtaacatgtggctcgcctctacgaggtgctgggtcaaactgcaagaaagagtattttagagtatcgtcaagttccatgattgcagcttggttaccacaacgataacaatagtttggagcactgaaaatcgttactacattccggtcatggcaccagttatatccctccatcactagctggtgagctctagacaccaacgtgaggccattggcatgattaaatgtctcagaaatatcttgcccaaaggtgtaaccagctcctcgaggagatataccccaaccaccacggtcatctggatctgaccacagcaagtcacacattggaccctaaaaaataactcatggggaacttcttgtaggcgatcaagtgctctgatatgatccagtgtatctatagatggcgagagaccaccatgtagacagaagatctgcccatccaccaaggcagtgagaggaagatagtcaaaaagatctgtaaaatatttccaaacatttgcatttccatattttcttaaacattcatcatagaaaccataaacttgtgtgatctgtctgctctcatgattccctcgaagaatggtgatgcgttcacggtaacgaaccttaagagctacaagcagtgtaactgtttcaactgaataatatcctctgtcaacataatctcccataaacaagtaatttgtatctggtgatttgccaccaattctaaacagttccatgagatcatgaaattgcccatgcacatctccacagacagtaactggacatcgaacctcttgcacgttggattcttttgtcaggatttctttagccttgatttctggagaagatcgcttggtgagtttaatacaaaccaccaaggggtactaaagctgtgtgacctttaggtatgttctgggatacggcctaacaagactgcctttgggggatcctctgggcagctctggacctaactaggcctgggtaccagcggcaagactcttactcagcccaccggagaggcccaggctccattcccaagccgcagaatccaagccagctcaccctcaaaaccgtccctgacgatgacccacagggtctccgctccccctgccacctcgtctggcgccaaggccggctgactcaaaagcccaggagtcgagtgaacggcgccatttt

SEQ ID NO: 15554 - RNA, 3401 nt, Homo sapiens
  source 1..3401: mol_type = other RNA
gctgggattacaggcatgagccactgtgccaggcctgttcttagggaaagctttttaggtttattaatgaaaatcctaatgttactaattgagacatcagttaacacccaacttagtgattcccatccaaccataattatgtatttttcaagaaaatacataatttactaacacattttccttaccatagccattttcaaaagaaggtagggtactaacactttccagtttagatggccaaagcccggtcagtctctataattaaacaattattttaaaccctagttatgctaaaaccaagctattcttatcacaagtcccattctgctaaccacaaaatttagagaatttgtacctggaagataccaccacgtgtcaattacaatatacgtattccttggtcaattctgatatcacaggaccggaaaaaatagctgcttggtgtctagattgtttgggtattaaaaccactgcacatggataagctatttgttcagtcggagagaaagggcatagagtgacagagcaacaaaaagacacacagagaatgtatttcttgtgaaagaaaagaatgaaatgaaatgaaatgtagaaaccctaatggccttttgctttggaaaattaactccacaagccactaaaaatactatcaattagatcagaaaagacattcggtatgtatgtgttcctcaagcattttagaaaggggatatgctataacttccctgttggttccagattcaacacagcacaaagcaagaaaacttttatttactacactcacaagtatgattaagtgttcctgtttactctggtaggttaaaatatcaaatattagttcccacagaagaacttttttttaaacatctaatcctattcgaaggataaaaggggaaaaactcattaaatgttgaacactgccactttaagtaccatttttgtcttcgggtgaatgtacataagactaaatcatgatccaacaatagttttctatttggtttcactagtatcactcaaagaacttgacacaggctaatgctttaacactttcttatctgagacaaatttaactctaagaacatatgactcaacaatgtacaaagatttaagaatttgccaatctgtcaatcattttaaagagtccatataatatacacatagcaatataatattcataaccagaaactgcactaagtaaacacatcatttagtttaagctctacctgaaaacatgctgttttattaaaacaaaacccaaagacttaaatctcaagttatatggttttacaattaagtcttactgaagcagcacagatttcctttcttacaaacaagttaatatgcaggaagaacccacaaagtgcacaccaacaatgtgacaaattgtaatatgtgaaatacaaataaatcctgaagttaatctgaagaatgtcaaggagttaccagagaggttatgtagtgcccttgatttttattttacctacaagtctacaaattctaaaatttactcaattgatttaacttttttaataaacagcaccagtcttgcccattgatacaattaaaatttgaccttctcagttcttagttcacaagtttattatgaaaaacactgcagtgctcttgtgcagtcacatcgtcttacaggaaggggaaaaaacagttctgttcaaaacaactcaccaggttctgacaataacaaagaacaacatggggctgagatttgagtagggaataaactgagtgcagacaaatcatataattaaattaaacggtatccctgaaaataaaaagaacaatttcaaaactcacaagtagaagggaggccttggtaattatttttaaaaatgttcattaagctccaatgattgtttgctgctatccttatctacagtcatgctgagtaaagctatagctaaatggaagttaaattgtattcacgaggtgttaatgtttacatcttattatctgcagtctctcagagaaagcaaaagtaactacaaatagcgctatgccagaaactggtttcttgaccaacaatgtcgcttcagcatgcaatgaactggttcattctaaagtggtcacggctgttgatgacaagaggctttgtatttttatatggcacatcttttggtccatgtgaaaacaagttttttgaatgttaactattttctgacactttggagttactgttgctcttcccatttccattaggtcgatatatggttcatggcaatactgtacaagtttaaaatttcattacaggaagtagtctggggtacgacgagtaacatgtggctcgcctctacgaggtgctgggtcaaactgcaagaaagagtattttagagtatcgtcaagttccatgattgcagcttggttaccacaacgataacaatagtttggagcactgaaaatcgttactacattccggtcatggcaccagttatatccctccatcactagctggtgagctctagacaccaacgtgaggccattggcatgattaaatgtctcagaaatatcttgcccaaaggtgtaaccagctcctcgaggagatataccccaaccaccacggtcatctggatctgaccacagcaagtcacacattggaccctcatggggaacttcttgtaggcgatcaagtgctctgatatgatccagtgtatctatagatggcgagagaccaccatgtagacagaagatctgcccatccaccaaggcagtgagaggaagatagtcaaaaagatctgtaaaatatttccaaacatttgcatttccatattttcttaaacattcatcatagaaaccataaacttgtgtgatctgtctgctctcatgattccctcgaagaatggtgatgcgttcacggtaacgaaccttaagagctacaagcagtgtaactgtttcaactgaataatatcctctgtcaacataatctcccataaacaagtaatttgtatctggtgatttgccaccaattctaaacagttccatgagatcatgaaattgcccatgcacatctccacagacagtaactggacatcgaacctcttgcacgttggattcttttgtcaggatttctttagccttctcgcagaggctcttgacctgggactcggacagctgcttgcactcgttcagctgctcgatccactggtccagctccttggtgaacaccttctcgtccatgatgccacccgccccagccggctgccgctccgcgctgctcccgcgccgccgcccgcacacgggcctacacgcacacgccgccgccggttcctcgtgtacttctggcggctgttgaggctggcgctggcccgctggctctcaccgcagtactcggccgtcggccgctgcgcctcctcctccgctcgctgaggctccagagctcggctctctgt

SEQ ID NO: 15555 - RNA, 3433 nt, Homo sapiens
  source 1..3433: mol_type = other RNA
gctgggattacaggcatgagccactgtgccaggcctgttcttagggaaagctttttaggtttattaatgaaaatcctaatgttactaattgagacatcagttaacacccaacttagtgattcccatccaaccataattatgtatttttcaagaaaatacataatttactaacacattttccttaccatagccattttcaaaagaaggtagggtactaacactttccagtttagatggccaaagcccggtcagtctctataattaaacaattattttaaaccctagttatgctaaaaccaagctattcttatcacaagtcccattctgctaaccacaaaatttagagaatttgtacctggaagataccaccacgtgtcaattacaatatacgtattccttggtcaattctgatatcacaggaccggaaaaaatagctgcttggtgtctagattgtttgggtattaaaaccactgcacatggataagctatttgttcagtcggagagaaagggcatagagtgacagagcaacaaaaagacacacagagaatgtatttcttgtgaaagaaaagaatgaaatgaaatgaaatgtagaaaccctaatggccttttgctttggaaaattaactccacaagccactaaaaatactatcaattagatcagaaaagacattcggtatgtatgtgttcctcaagcattttagaaaggggatatgctataacttccctgttggttccagattcaacacagcacaaagcaagaaaacttttatttactacactcacaagtatgattaagtgttcctgtttactctggtaggttaaaatatcaaatattagttcccacagaagaacttttttttaaacatctaatcctattcgaaggataaaaggggaaaaactcattaaatgttgaacactgccactttaagtaccatttttgtcttcgggtgaatgtacataagactaaatcatgatccaacaatagttttctatttggtttcactagtatcactcaaagaacttgacacaggctaatgctttaacactttcttatctgagacaaatttaactctaagaacatatgactcaacaatgtacaaagatttaagaatttgccaatctgtcaatcattttaaagagtccatataatatacacatagcaatataatattcataaccagaaactgcactaagtaaacacatcatttagtttaagctctacctgaaaacatgctgttttattaaaacaaaacccaaagacttaaatctcaagttatatggttttacaattaagtcttactgaagcagcacagatttcctttcttacaaacaagttaatatgcaggaagaacccacaaagtgcacaccaacaatgtgacaaattgtaatatgtgaaatacaaataaatcctgaagttaatctgaagaatgtcaaggagttaccagagaggttatgtagtgcccttgatttttattttacctacaagtctacaaattctaaaatttactcaattgatttaacttttttaataaacagcaccagtcttgcccattgatacaattaaaatttgaccttctcagttcttagttcacaagtttattatgaaaaacactgcagtgctcttgtgcagtcacatcgtcttacaggaaggggaaaaaacagttctgttcaaaacaactcaccaggttctgacaataacaaagaacaacatggggctgagatttgagtagggaataaactgagtgcagacaaatcatataattaaattaaacggtatccctgaaaataaaaagaacaatttcaaaactcacaagtagaagggaggccttggtaattatttttaaaaatgttcattaagctccaatgattgtttgctgctatccttatctacagtcatgctgagtaaagctatagctaaatggaagttaaattgtattcacgaggtgttaatgtttacatcttattatctgcagtctctcagagaaagcaaaagtaactacaaatagcgctatgccagaaactggtttcttgaccaacaatgtcgcttcagcatgcaatgaactggttcattctaaagtggtcacggctgttgatgacaagaggctttgtatttttatatggcacatcttttggtccatgtgaaaacaagttttttgaatgttaactattttctgacactttggagttactgttgctcttcccatttccattaggtcgatatatggttcatggcaatactgtacaagtttaaaatttcattacaggaagtagtctggggtacgacgagtaacatgtggctcgcctctacgaggtgctgggtcaaactgcaagaaagagtattttagagtatcgtcaagttccatgattgcagcttggttaccacaacgataacaatagtttggagcactgaaaatcgttactacattccggtcatggcaccagttatatccctccatcactagctggtgagctctagacaccaacgtgaggccattggcatgattaaatgtctcagaaatatcttgcccaaaggtgtaaccagctcctcgaggagatataccccaaccaccacggtcatctggatctgaccacagcaagtcacacattggaccctcatggggaacttcttgtaggcgatcaagtgctctgatatgatccagtgtatctatagatggcgagagaccaccatgtagacagaagatctgcccatccaccaaggcagtgagaggaagatagtcaaaaagatctgtaaaatatttccaaacatttgcatttccatattttcttaaacattcatcatagaaaccataaacttgtgtgatctgtctgctctcatgattccctcgaagaatggtgatgcgttcacggtaacgaaccttaagagctacaagcagtgtaactgtttcaactgaataatatcctctgtcaacataatctcccataaacaagtaatttgtatctggtgatttgccaccaattctaaacagttccatgagatcatgaaattgcccatgcacatctccacagacagtaactggacatcgaacctcttgcacgttggattcttttgtcaggatttctttagccttgatttctggagaagatcgcttggtgagtttaatacaaaccaccaaggggtactaaagctgtgtgacctttaggtatgttctgggatacggcctaacaagactgcctttgggggatcctctgggcagctctggacctaactaggcctgggtaccagcggcaagactcttactcagcccaccggagaggcccaggctccattcccaagccgcagaatccaagccagctcaccctcaaaaccgtccctgacgatgacccacagggtctccgctccccctgccacctcgtctggcgccaaggccggctgactcaaaagcccaggagtcgagtgaacggcgccatttt

SEQ ID NO: 15556 - RNA, 1793 nt, Homo sapiens
  source 1..1793: mol_type = other RNA
gctgggattacaggcatgagccactgtgccaggctgagaattcaattattgactgtggcagtttgaaaattttttctcaatttttttattttgataaatttcaaaccttcagagaaatttcaagaatagtgtagtgaaaggtcatataaccttcacctatcttcatcaattttttttaaattgtaattattattttttatagagacagcgtctccctatgtttcccaggctggtctcaaactgctgggctcaaggaatcctacctcctcagcctcccagagggctgggattacaggcatgagccacccaccatacctggcccaccaattgttaatattttgccacatttgtgttctctctttcatatacaggcacagacacatatatacatatttttttttctgaactatttgaaagttagttgcaaacatgacacttttatctctaaatactgtacttcagcatatgtcttctgagtacaaggacattcccccatataaccacaataatcaaacccaggaaatttaactattacctaagactattatctaactatagtccatattcaaatttccccaagtatctagtaatgtcctctatacctgttaacttattgaggatcttgcattgcatttgtctcttttagtctagatttaagtacctttgttttgtcattatgacattgactattttgaagagttgaagtcaggttccatcctcccatccctatcgcaatgtccttcaatttgtatctgtctgattctttctttctatttttttgagacagggtctcactctgttgtccaggctggaatgcagcagtgcaatcttggctcactgcaacttcggcctcctggtctcaagcgatcctcccacctcagtctctcaagtagctaggactatagtcacatgccaccatgcccagctaatttttgtattttttgtagagatggagttttgccatgttgcccaggttggtcttgaactcctaggctcaagtagtctacatgtctcagccttccaaagtgctgggattacaggcatgagccactgtgcccagcctgattgtttctttatgatgagactcaggttaaatatttttggcagaatattacaaataagtcatgtttcaatgccaccttttataaatgtttcttatccttctcttttaaatgtgtgaagccaggaataataaaaagtctaataatcttattttcaaatatctagcaggtcatttattggcaagtgactcttgtcatcacgtcatgattgaggcagtaggctatttatacagatcagttgatttaagggtgatccacctgggatcttctcattcatcaatccatggaatccatggaatcctgcagtgagtttctgtttcatgttccaaacagaaatatgcttctggttattcatgctatatatatgacctcttgacaacttttgatcttttgcagccttctgagagaaattgagtggatccggagccggagatattggcctcaaggtatgagccagcaacattctgagggttctaggaatggcttctcattatgggagcacttggttaaattaaactaccacagtgctcagagttctaatacagtgagctctgcaatgtgcatgaatgcagataaattacacagggctagaagaatggacttggcacctcagacaatttcagataaatcaaaatgtgctcctcatcattccatcccatgtggcctgcgcgccaccacaccacacggccacccccgcgccaccctgaaattgaccgcagcaggctgggcgtg

SEQ ID NO: 15557 - RNA, 2933 nt, Homo sapiens
  source 1..2933: mol_type = other RNA
gctgggattacaggcatgagccactgtgcccagacagtaaaatacttcttatactcagtaagtaattctgtctatagttaataattaaattaaacccatattcaaattatagaaagcatttttgcccaccaaatcatcttaccatttctaatatactctctctctcttgaatcaacttattaaataactcatgtaatctgcatcctcagctccagtgttcattaaaaaggaaaaaaacccactattttaaagcaaaatggtggctccttctcagtagcttttttttttttcttttttttgagacagactctcactgtgtcgcccaggttggagtgcagtggcgtgatctccacttactgcaacctctgcctcccgggttcaagtgattctcctgcctcagtctcccgagtagctgggactacaggtgcgtgccaccacacccagctaatttttgtatttttggtagagacggggtttcaccatgttggtcaggatagtctcaatctcttgaccttgtgatccacctgcctcagcctcccaaactgctaggattacaggcgtgagccactgcgccaggccttctcagcagctcttgtgggaacacagaaagggaattcaaaatttggctacctctcccactcatgtgatcagggaagaataggcttatgagagacctaaaaaaatcttccgagcagccttggatttaaagtcatagcgctgtttaaaataaagtaatatggcaatctggaatgtctccaagaaaagtcattttgttctgtcactgacatctgtactatttgtttgaatgttgtttttgtaaacagttgtagattaaagaagtttttacagatcaatgagtaaaatgttcatttaataactttctaactgtatacagtatatgcttgatagttcaaaattctccaaatgtagatattatacaataattattttaaattattaaatgagtatttaatccttttaaattacattttgaaaatttaatggcaattacacacaaattttaatttaaaataatattaaggacttaatctgatttacagaaatgaaatgcaatgaagagattaagggctaacctccattactataaaattctctggctaccatctagcacaggagcaactggattgctttcagcagtcttgaagcactaaaatatcttaaaattcatatggagaaatagtatgtatctctacattaaatttagatttgatatttattctctgacagatcagacccagaatattaatttttatgtaattgaaccaaaaacatttagcaatccttcatttagtaatcttttgtataaatataaaaatctctgataagtgaaatgttttttcaaattatacttctatttttcacagctttataggtaattataattttcaaactttaaatatttcatgtgatttgatatatctgtacagaaagagtaagataaaaacatttaataagattaaatctaatttgcaaaaattggtatctgacatttgttgtgtgctcttgcaaagagtgcataggacatttctgcagcaatcaaaaaggtaaaatctttttaaactcagatttcaagtttcctctaatattccttctaatcctaatccctggaaatactttcaagttttgatttctagatgcaatgtgttttgttacatatacacatgtcttatccttaaacttttaaaaaacagtatgatcagattcagcatgatgatatcttctcagactctgtagaagtcctctgtgcaagattaatgtcgagattcctagtgccccatcgtgaaaaaccagttaaagatagtatacaactatgctttagtgggatttcctgcaggtttgggatcataaccatacaaaaaagtagctgttattacaaggatggctccaaggaaaaagacacaagctgaatatttcttatccacactgattgttttgtttcttttaagattttctcaaagtaaaccccagcaaagccacttgaaaaacatgctgtgagaactgccatgagtcctacaaattgagaaccagctgaaagttccttagaatcaagctgagaatctgagggccactgtacaaaagcaactcctgtcatcaaaattactagggacagccactggtatacacccaattttttactaagcatagacacagaaaataatgctgttgtaagaatttttaactgatacgtgacctgataagtagctgcatctagatttgatagtgccacatacagtaaattattctgaagagtatagatccctgatggaatagcaagtttaagtgtttccataggtttattaagaatttcatcatgtagtactcgattcagtgctcttagactacatttgctgtctttgtagaccaataaaatgcaggccattatcttcaaaagttcagcaacaaccactgctgtagaagatagataacgaggtccttcttcttttaaagttctggaataacgcattgttagaaccaaactggtagtctgaaagaccaaaattcccagggaaacgtattttaggttggcgaacattgttttatcttcatttgccaagggcagcctttccatttctttaagttcctgcggcttcttgagctccaggtgctggtcgggtgcatctgtgcctaccacagggctcaacaccgagcgagagctcatgggatgttcactgaaggaatgacgggccccagccgggcccacccgtcactagctccgcacgcaccaggcgctgaggcacacactgccgtcttcattcgcttgacacacccctctcctcgggccttttttcctcctccacccagtacattccgcacgtcgtccgtcggagttacaacgtgtcacctcatctgctcccacccctacttagctagcactgtatttcaggtcttcgataccgtccccttcaccccta

SEQ ID NO: 15558 - RNA, 2739 nt, Homo sapiens
  source 1..2739: mol_type = other RNA
gctgggattacaggcatgagccactgtgcccagacagtaaaatacttcttatactcagtaagtaattctgtctatagttaataattaaattaaacccatattcaaattatagaaagcatttttgcccaccaaatcatcttaccatttctaatatactctctctctcttgaatcaacttattaaataactcatgtaatctgcatcctcagctccagtgttcattaaaaaggaaaaaaacccactattttaaagcaaaatggtggctccttctcagtagcttttttttttttcttttttttgagacagactctcactgtgtcgcccaggttggagtgcagtggcgtgatctccacttactgcaacctctgcctcccgggttcaagtgattctcctgcctcagtctcccgagtagctgggactacaggtgcgtgccaccacacccagctaatttttgtatttttggtagagacggggtttcaccatgttggtcaggatagtctcaatctcttgaccttgtgatccacctgcctcagcctcccaaactgctaggattacaggcgtgagccactgcgccaggccttctcagcagctcttgtgggaacacagaaagggaattcaaaatttggctacctctcccactcatgtgatcagggaagaataggcttatgagagacctaaaaaaatcttccgagcagccttggatttaaagtcatagcgctgtttaaaataaagtaatatggcaatctggaatgtctccaagaaaagtcattttgttctgtcactgacatctgtactatttgtttgaatgttgtttttgtaaacagttgtagattaaagaagtttttacagatcaatgagtaaaatgttcatttaataactttctaactgtatacagtatatgcttgatagttcaaaattctccaaatgtagatattatacaataattattttaaattattaaatgagtatttaatccttttaaattacattttgaaaatttaatggcaattacacacaaattttaatttaaaataatattaaggacttaatctgatttacagaaatgaaatgcaatgaagagattaagggctaacctccattactataaaattctctggctaccatctagcacaggagcaactggattgctttcagcagtcttgaagcactaaaatatcttaaaattcatatggagaaatagtatgtatctctacattaaatttagatttgatatttattctctgacagatcagacccagaatattaatttttatgtaattgaaccaaaaacatttagcaatccttcatttagtaatcttttgtataaatataaaaatctctgataagtgaaatgttttttcaaattatacttctatttttcacagctttataggtaattataattttcaaactttaaatatttcatgtgatttgatatatctgtacagaaagagtaagataaaaacatttaataagattaaatctaatttgcaaaaattggtatctgacatttgttgtgtgctcttgcaaagagtgcataggacatttctgcagcaatcaaaaaggtaaaatctttttaaactcagatttcaagtttcctctaatattccttctaatcctaatccctggaaatactttcaagttttgatttctagatgcaatgtgttttgttacatatacacatgtcttatccttaaacttttaaaaaacagtatgatcagattcagcatgatgatatcttctcagactctgtagaagtcctctgtgcaagattaatgtcgagattcctagtgccccatcgtgaaaaaccagttaaagatagtatacaactatgctttagtgggatttcctgcaggtttgggatcataaccatacaaaaaagtagctgttattacaaggatggctccaaggaaaaagacacaagctgaatatttcttatccacactgattgttttgtttcttttaagattttctcaaagtaaaccccagcaaagccacttgaaaaacatgctgtgagaactgccatgagtcctacaaattgagaaccagctgaaagttccttagaatcaagctgagaatctgagggccactgtacaaaagcaactcctgtcatcaaaattactagggacagccactggtatacacccaattttttactaagcatagacacagaaaataatgctgttgtaagaatttttaactgatacgtgacctgataagtagctgcatctagatttgatagtgccacatacagtaaattattctgaagagtatagatccctgatggaatagcaagtttaagtgtttccataggtttattaagaatttcatcatgtagtactcgattcagtgctcttagactacatttgctgtctttgtagaccaataaaatgcaggccattatcttcaaaagttcagcaacaaccactgctgtagaagatagataacgaggtccttcttcttttaaagttctggaataacgcattgttagaaccaaactggtagtctgaaagaccaaaattcccagggaaacgtattttaggttggcgaacattgttttatcttcatttgcctcccgcgcagctcgaccggctgagcccaccaccgggggccgcggttcagctccgccgggcgccccaggctgccgagtccgctgggtcctacgcgaccgctgacccgcagcgccgccggctcccgtcgccgtagccaccgccagctcggtgcagcccaggcgtttcc

SEQ ID NO: 15559 - RNA, 4330 nt, Homo sapiens
  source 1..4330: mol_type = other RNA
gctgggattacaggcatgagccactgtgcccagacagtaaaatacttcttatactcagtaagtaattctgtctatagttaataattaaattaaacccatattcaaattatagaaagcatttttgcccaccaaatcatcttaccatttctaatatactctctctctcttgaatcaacttattaaataactcatgtaatctgcatcctcagctccagtgttcattaaaaaggaaaaaaacccactattttaaagcaaaatggtggctccttctcagtagcttttttttttttcttttttttgagacagactctcactgtgtcgcccaggttggagtgcagtggcgtgatctccacttactgcaacctctgcctcccgggttcaagtgattctcctgcctcagtctcccgagtagctgggactacaggtgcgtgccaccacacccagctaatttttgtatttttggtagagacggggtttcaccatgttggtcaggatagtctcaatctcttgaccttgtgatccacctgcctcagcctcccaaactgctaggattacaggcgtgagccactgcgccaggccttctcagcagctcttgtgggaacacagaaagggaattcaaaatttggctacctctcccactcatgtgatcagggaagaataggcttatgagagacctaaaaaaatcttccgagcagccttggatttaaagtcatagcgctgtttaaaataaagtaatatggcaatctggaatgtctccaagaaaagtcattttgttctgtcactgacatctgtactatttgtttgaatgttgtttttgtaaacagttgtagattaaagaagtttttacagatcaatgagtaaaatgttcatttaataactttctaactgtatacagtatatgcttgatagttcaaaattctccaaatgtagatattatacaataattattttaaattattaaatgagtatttaatccttttaaattacattttgaaaatttaatggcaattacacacaaattttaatttaaaataatattaaggacttaatctgatttacagaaatgaaatgcaatgaagagattaagggctaacctccattactataaaattctctggctaccatctagcacaggagcaactggattgctttcagcagtcttgaagcactaaaatatcttaaaattcatatggagaaatagtatgtatctctacattaaatttagatttgatatttattctctgacagatcagacccagaatattaatttttatgtaattgaaccaaaaacatttagcaatccttcatttagtaatcttttgtataaatataaaaatctctgataagtgaaatgttttttcaaattatacttctatttttcacagctttataggtaattataattttcaaactttaaatatttcatgtgatttgatatatctgtacagaaagagtaagataaaaacatttaataagattaaatctaatttgcaaaaattggtatctgacatttgttgtgtgctcttgcaaagagtgcataggacatttctgcagcaatcaaaaaggtaaaatctttttaaactcagatttcaagtttcctctaatattccttctaatcctaatccctggaaatactttcaagttttgatttctagatgcaatgtgttttgttacatatacacatgtcttatccttaaacttttaaaaaacagtatgatcagattcagcatgatgatatcttctcagactctgtagaagtcctctgtgcaagattaatgtcgagattcctagtgccccatcgtgaaaaaccagttaaagatagtatacaactatgctttagtgggatttcctgcaggtttgggatcataaccatacaaaaaagtagctgttattacaaggatggctccaaggaaaaagacactgaagaacaactactatccaggtcagtcggttatatccctgaaaaaatccattctttgataccagttctccatcataaatgtatacacccattaatccaaatatacttccaaagaaaccaagctgaatatttcttatccacactgattgttttgtttcttttaagattttctcaaagtaaaccccagcaaagccacttgaaaaacatgctgtgagaactgccatgagtcctacaaattgagaaccagctgaaagttccttagaatcaagctgagaatctgagggccactgataagtagctgcatctagatttgatagtgccacatacagtaaattattctgaagagtatagatccctgatggaatagcaagtttaagtgtttccataggtttattaagaatttcatcatgtagtactcgattcagtgctcttagactacatttgctgtctttgtagaccaataaaatgcaggccattatcttcaaaagttcagcaacaaccactgctgtagaagatagataacgaggtccttcttcttttaaagttctggaataacgcattgttagaaccaaactggtagtctgaaagaccaaaattcccagggaaacgtattttaggttggcgaacattgttttatcttcatttgcctcccgcgcagctcgaccggctgagcccaccaccgggggccgcggttcagctccgccgggcgccccaggctgccgagtccgctgggtcctacgcgaccgctgacccgcagcgccgccggctcccgtcgccgtagccaccgccagctcggtgcagcccaggcgtttccgggttcccgcggtcccgtcccccaaatgctccggcttccgcctcggctctggcaaatgccgttcccggctcggctctggcagccccagctcggcacttggcagctctgtccctaaggcgacgcacctgggctgctctgctggcagcccctggttcctgcttcaccgtcgcgtggaggcctggggcactgctttctgctacacctctcctaggagcgcgaaacagatggagtgacactcgtcgagggcctctgcgggactgtctgtttgcagagggtgccaaggtgtccactgcgtaaggaagggcaaagtcctttggggcaaagaaccctgagaggaacggggagatggattttgaaagcaaacgaaccctctcctaaaagtgactgtcactgacctgaaaacaaccagattagctatggcaaaggctgccaaccaaccagtggtctgcaagaaggcttgttcttccacttcacccaccctgactgagatcttgagactgaaggaaacccaaagccgtaccaccaatgggcctagtgtcatcaaccgggagaggaaaaagaaaactgggcccagaggattgcagagttatgagggaccaaccccttcctggctgcatggatcacagcattaccttttaaaagtgttccagtagctgtgttggaaaccctctaaccacggcagcccattcaggtgatgaacaggctgaaatcagtacttcaggttcagctggattatcaaataagcgaataggattatctctttttgttaactcagggctgctataaattaagcctatgtctctttatattgcaaatgattaaaaccatgtccaagagagacatacttagaaaaaaagtgatattgaagaaaaataagtaactgtattagagtagaataactggttttaaaattttctgcaatacagtcttgagaaaattcctggatggtaaaatacatattagatcttaatacatgcccagttttttttgaaaccaaaatgtgcctgttagatgatgataacagcatgcctcgttttattgtgatttgctttattgctcttcacagacattgcttttgtttttttgttttttttttttacaaattgaaggtttgtggcaaccttgcctcaagcacatctattggtgccatttttccaacagcatgtgctcactttgtgtctctgtgtcacataatattcaataatttttgcaatatttaaatttgttcatcattattatatctggtatagtgctttgtgatcaatgatctttgatgttactatggtaattgttttggggtgctgatatggtttggctgtgtccccacccaaatctcaacttgaactgtatctcccagaattcccacgtgttgagggagagacctagggggagataattgaatcatgggggccagtctttcctgtgctattctcatgatagtgaataagtctcatgaaatccgatgggtttatctggggtttctgattttgcttcttcctcatttttctcttgctgcagccatgtaagcaagtacctttcacctcccgccatgattctgaggcctcccccgccatgtggaactgtaggtccaatta

SEQ ID NO: 15560 - RNA, 3042 nt, Homo sapiens
  source 1..3042: mol_type = other RNA
gctgggattacaggcatgagccactgtgcccagacagtaaaatacttcttatactcagtaagtaattctgtctatagttaataattaaattaaacccatattcaaattatagaaagcatttttgcccaccaaatcatcttaccatttctaatatactctctctctcttgaatcaacttattaaataactcatgtaatctgcatcctcagctccagtgttcattaaaaaggaaaaaaacccactattttaaagcaaaatggtggctccttctcagtagcttttttttttttcttttttttgagacagactctcactgtgtcgcccaggttggagtgcagtggcgtgatctccacttactgcaacctctgcctcccgggttcaagtgattctcctgcctcagtctcccgagtagctgggactacaggtgcgtgccaccacacccagctaatttttgtatttttggtagagacggggtttcaccatgttggtcaggatagtctcaatctcttgaccttgtgatccacctgcctcagcctcccaaactgctaggattacaggcgtgagccactgcgccaggccttctcagcagctcttgtgggaacacagaaagggaattcaaaatttggctacctctcccactcatgtgatcagggaagaataggcttatgagagacctaaaaaaatcttccgagcagccttggatttaaagtcatagcgctgtttaaaataaagtaatatggcaatctggaatgtctccaagaaaagtcattttgttctgtcactgacatctgtactatttgtttgaatgttgtttttgtaaacagttgtagattaaagaagtttttacagatcaatgagtaaaatgttcatttaataactttctaactgtatacagtatatgcttgatagttcaaaattctccaaatgtagatattatacaataattattttaaattattaaatgagtatttaatccttttaaattacattttgaaaatttaatggcaattacacacaaattttaatttaaaataatattaaggacttaatctgatttacagaaatgaaatgcaatgaagagattaagggctaacctccattactataaaattctctggctaccatctagcacaggagcaactggattgctttcagcagtcttgaagcactaaaatatcttaaaattcatatggagaaatagtatgtatctctacattaaatttagatttgatatttattctctgacagatcagacccagaatattaatttttatgtaattgaaccaaaaacatttagcaatccttcatttagtaatcttttgtataaatataaaaatctctgataagtgaaatgttttttcaaattatacttctatttttcacagctttataggtaattataattttcaaactttaaatatttcatgtgatttgatatatctgtacagaaagagtaagataaaaacatttaataagattaaatctaatttgcaaaaattggtatctgacatttgttgtgtgctcttgcaaagagtgcataggacatttctgcagcaatcaaaaaggtaaaatctttttaaactcagatttcaagtttcctctaatattccttctaatcctaatccctggaaatactttcaagttttgatttctagatgcaatgtgttttgttacatatacacatgtcttatccttaaacttttaaaaaacagtatgatcagattcagcatgatgatatcttctcagactctgtagaagtcctctgtgcaagattaatgtcgagattcctagtgccccatcgtgaaaaaccagttaaagatagtatacaactatgctttagtgggatttcctgcaggtttgggatcataaccatacaaaaaagtagctgttattacaaggatggctccaaggaaaaagacactgaagaacaactactatccaggtcagtcggttatatccctgaaaaaatccattctttgataccagttctccatcataaatgtatacacccattaatccaaatatacttccaaagaaaccaagctgaatatttcttatccacactgattgttttgtttcttttaagattttctcaaagtaaaccccagcaaagccacttgaaaaacatgctgtgagaactgccatgagtcctacaaattgagaaccagctgaaagttccttagaatcaagctgagaatctgagggccactgtacaaaagcaactcctgtcatcaaaattactagggacagccactggtatacacccaattttttactaagcatagacacagaaaataatgctgttgtaagaatttttaactgatacgtgacctgataagtagctgcatctagatttgatagtgccacatacagtaaattattctgaagagtatagatccctgatggaatagcaagtttaagtgtttccataggtttattaagaatttcatcatgtagtactcgattcagtgctcttagactacatttgctgtctttgtagaccaataaaatgcaggccattatcttcaaaagttcagcaacaaccactgctgtagaagatagataacgaggtccttcttcttttaaagttctggaataacgcattgttagaaccaaactggtagtctgaaagaccaaaattcccagggaaacgtattttaggttggcgaacattgttttatcttcatttgccaagggcagcctttccatttctttaagttcctgcggcttcttgagctccaggtgctggtcgggtgcatctgtgcctaccacagggctcaacaccgagcgagagctcatgggatgttcactgaaggaatgacgggccccagccgggcccacccgtcactagctccgcacgcaccaggcgctgaggcacacactgccgtcttcattcgcttgacacacccctctcctcgggccttttttcctcctccacccagtacattccgcacgtcgtccgtcggagttacaacgtgtcacctcatctgctcccacccctacttagctagcactgtatttcaggtcttcgataccgtcccc

SEQ ID NO: 15561 - RNA, 2823 nt, Homo sapiens
  source 1..2823: mol_type = other RNA
gctgggattacaggcatgagccactgtgcccagacagtaaaatacttcttatactcagtaagtaattctgtctatagttaataattaaattaaacccatattcaaattatagaaagcatttttgcccaccaaatcatcttaccatttctaatatactctctctctcttgaatcaacttattaaataactcatgtaatctgcatcctcagctccagtgttcattaaaaaggaaaaaaacccactattttaaagcaaaatggtggctccttctcagtagcttttttttttttcttttttttgagacagactctcactgtgtcgcccaggttggagtgcagtggcgtgatctccacttactgcaacctctgcctcccgggttcaagtgattctcctgcctcagtctcccgagtagctgggactacaggtgcgtgccaccacacccagctaatttttgtatttttggtagagacggggtttcaccatgttggtcaggatagtctcaatctcttgaccttgtgatccacctgcctcagcctcccaaactgctaggattacaggcgtgagccactgcgccaggccttctcagcagctcttgtgggaacacagaaagggaattcaaaatttggctacctctcccactcatgtgatcagggaagaataggcttatgagagacctaaaaaaatcttccgagcagccttggatttaaagtcatagcgctgtttaaaataaagtaatatggcaatctggaatgtctccaagaaaagtcattttgttctgtcactgacatctgtactatttgtttgaatgttgtttttgtaaacagttgtagattaaagaagtttttacagatcaatgagtaaaatgttcatttaataactttctaactgtatacagtatatgcttgatagttcaaaattctccaaatgtagatattatacaataattattttaaattattaaatgagtatttaatccttttaaattacattttgaaaatttaatggcaattacacacaaattttaatttaaaataatattaaggacttaatctgatttacagaaatgaaatgcaatgaagagattaagggctaacctccattactataaaattctctggctaccatctagcacaggagcaactggattgctttcagcagtcttgaagcactaaaatatcttaaaattcatatggagaaatagtatgtatctctacattaaatttagatttgatatttattctctgacagatcagacccagaatattaatttttatgtaattgaaccaaaaacatttagcaatccttcatttagtaatcttttgtataaatataaaaatctctgataagtgaaatgttttttcaaattatacttctatttttcacagctttataggtaattataattttcaaactttaaatatttcatgtgatttgatatatctgtacagaaagagtaagataaaaacatttaataagattaaatctaatttgcaaaaattggtatctgacatttgttgtgtgctcttgcaaagagtgcataggacatttctgcagcaatcaaaaaggtaaaatctttttaaactcagatttcaagtttcctctaatattccttctaatcctaatccctggaaatactttcaagttttgatttctagatgcaatgtgttttgttacatatacacatgtcttatccttaaacttttaaaaaacagtatgatcagattcagcatgatgatatcttctcagactctgtagaagtcctctgtgcaagattaatgtcgagattcctagtgccccatcgtgaaaaaccagttaaagatagtatacaactatgctttagtgggatttcctgcaggtttgggatcataaccatacaaaaaagtagctgttattacaaggatggctccaaggaaaaagacactgaagaacaactactatccaggtcagtcggttatatccctgaaaaaatccattctttgataccagttctccatcataaatgtatacacccattaatccaaatatacttccaaagaaaccaagctgaatatttcttatccacactgattgttttgtttcttttaagattttctcaaagtaaaccccagcaaagccacttgaaaaacatgctgtgagaactgccatgagtcctacaaattgagaaccagctgaaagttccttagaatcaagctgagaatctgagggccactgtacaaaagcaactcctgtcatcaaaattactagggacagccactggtatacacccaattttttactaagcatagacacagaaaataatgctgttgtaagaatttttaactgatacgtgacctgataagtagctgcatctagatttgatagtgccacatacagtaaattattctgaagagtatagatccctgatggaatagcaagtttaagtgtttccataggtttattaagaatttcatcatgtagtactcgattcagtgctcttagactacatttgctgtctttgtagaccaataaaatgcaggccattatcttcaaaagttcagcaacaaccactgctgtagaagatagataacgaggtccttcttcttttaaagttctggaataacgcattgttagaaccaaactggtagtctgaaagaccaaaattcccagggaaacgtattttaggttggcgaacattgttttatcttcatttgcctcccgcgcagctcgaccggctgagcccaccaccgggggccgcggttcagctccgccgggcgccccaggctgccgagtccgctgggtcctacgcgaccgctgacccgcagcgccgccggctcccgtcgccgt

SEQ ID NO: 15562 - RNA, 3054 nt, Homo sapiens
  source 1..3054: mol_type = other RNA
gctgggattacaggcatgagccactgtgcccagacagtaaaatacttcttatactcagtaagtaattctgtctatagttaataattaaattaaacccatattcaaattatagaaagcatttttgcccaccaaatcatcttaccatttctaatatactctctctctcttgaatcaacttattaaataactcatgtaatctgcatcctcagctccagtgttcattaaaaaggaaaaaaacccactattttaaagcaaaatggtggctccttctcagtagcttttttttttttcttttttttgagacagactctcactgtgtcgcccaggttggagtgcagtggcgtgatctccacttactgcaacctctgcctcccgggttcaagtgattctcctgcctcagtctcccgagtagctgggactacaggtgcgtgccaccacacccagctaatttttgtatttttggtagagacggggtttcaccatgttggtcaggatagtctcaatctcttgaccttgtgatccacctgcctcagcctcccaaactgctaggattacaggcgtgagccactgcgccaggccttctcagcagctcttgtgggaacacagaaagggaattcaaaatttggctacctctcccactcatgtgatcagggaagaataggcttatgagagacctaaaaaaatcttccgagcagccttggatttaaagtcatagcgctgtttaaaataaagtaatatggcaatctggaatgtctccaagaaaagtcattttgttctgtcactgacatctgtactatttgtttgaatgttgtttttgtaaacagttgtagattaaagaagtttttacagatcaatgagtaaaatgttcatttaataactttctaactgtatacagtatatgcttgatagttcaaaattctccaaatgtagatattatacaataattattttaaattattaaatgagtatttaatccttttaaattacattttgaaaatttaatggcaattacacacaaattttaatttaaaataatattaaggacttaatctgatttacagaaatgaaatgcaatgaagagattaagggctaacctccattactataaaattctctggctaccatctagcacaggagcaactggattgctttcagcagtcttgaagcactaaaatatcttaaaattcatatggagaaatagtatgtatctctacattaaatttagatttgatatttattctctgacagatcagacccagaatattaatttttatgtaattgaaccaaaaacatttagcaatccttcatttagtaatcttttgtataaatataaaaatctctgataagtgaaatgttttttcaaattatacttctatttttcacagctttataggtaattataattttcaaactttaaatatttcatgtgatttgatatatctgtacagaaagagtaagataaaaacatttaataagattaaatctaatttgcaaaaattggtatctgacatttgttgtgtgctcttgcaaagagtgcataggacatttctgcagcaatcaaaaaggtaaaatctttttaaactcagatttcaagtttcctctaatattccttctaatcctaatccctggaaatactttcaagttttgatttctagatgcaatgtgttttgttacatatacacatgtcttatccttaaacttttaaaaaacagtatgatcagattcagcatgatgatatcttctcagactctgtagaagtcctctgtgcaagattaatgtcgagattcctagtgccccatcgtgaaaaaccagttaaagatagtatacaactatgctttagtgggatttcctgcaggtttgggatcataaccatacaaaaaagtagctgttattacaaggatggctccaaggaaaaagacactggttggcacaaaatcttgaagccaaaaataggagatcaatgttgataatattatcgataaagaggttgcaaatccttttaaaatattatctgcatacttaataacagcagctattacaaggcctccaagtgcctgaagaacaactactatccaggtcagtcggttatatccctgaaaaaatccattctttgataccagttctccatcataaatgtatacacccattaatccaaatatacttccaaagaaaccaagctgaatatttcttatccacactgattgttttgtttcttttaagattttctcaaagtaaaccccagcaaagccacttgaaaaacatgctgtgagaactgccatgagtcctacaaattgagaaccagctgaaagttccttagaatcaagctgagaatctgagggccactgataagtagctgcatctagatttgatagtgccacatacagtaaattattctgaagagtatagatccctgatggaatagcaagtttaagtgtttccataggtttattaagaatttcatcatgtagtactcgattcagtgctcttagactacatttgctgtctttgtagaccaataaaatgcaggccattatcttcaaaagttcagcaacaaccactgctgtagaagatagataacgaggtccttcttcttttaaagttctggaataacgcattgttagaaccaaactggtagtctgaaagaccaaaattcccagggaaacgtattttaggttggcgaacattgttttatcttcatttgccaagggcagcctttccatttctttaagttcctgcggcttcttgagctccaggtgctggtcgggtgcatctgtgcctaccacagggctcaacaccgagcgagagctcatgggatgttcactgaaggaatgacgggccccagccgggcccacccgtcactagctccgcacgcaccaggcgctgaggcacacactgccgtcttcattcgcttgacacacccctctcctcgggccttttttcctcctccacccagtacattccgcacgtcgtccgtcggagttacaacgtgtcacctcatctgctcccacccctacttagctagcactgtatttcaggtcttcgataccgtcccct

SEQ ID NO: 15563 - RNA, 4464 nt, Homo sapiens
  source 1..4464: mol_type = other RNA
gctgggattacaggcatgagccactgtgcccagacagtaaaatacttcttatactcagtaagtaattctgtctatagttaataattaaattaaacccatattcaaattatagaaagcatttttgcccaccaaatcatcttaccatttctaatatactctctctctcttgaatcaacttattaaataactcatgtaatctgcatcctcagctccagtgttcattaaaaaggaaaaaaacccactattttaaagcaaaatggtggctccttctcagtagcttttttttttttcttttttttgagacagactctcactgtgtcgcccaggttggagtgcagtggcgtgatctccacttactgcaacctctgcctcccgggttcaagtgattctcctgcctcagtctcccgagtagctgggactacaggtgcgtgccaccacacccagctaatttttgtatttttggtagagacggggtttcaccatgttggtcaggatagtctcaatctcttgaccttgtgatccacctgcctcagcctcccaaactgctaggattacaggcgtgagccactgcgccaggccttctcagcagctcttgtgggaacacagaaagggaattcaaaatttggctacctctcccactcatgtgatcagggaagaataggcttatgagagacctaaaaaaatcttccgagcagccttggatttaaagtcatagcgctgtttaaaataaagtaatatggcaatctggaatgtctccaagaaaagtcattttgttctgtcactgacatctgtactatttgtttgaatgttgtttttgtaaacagttgtagattaaagaagtttttacagatcaatgagtaaaatgttcatttaataactttctaactgtatacagtatatgcttgatagttcaaaattctccaaatgtagatattatacaataattattttaaattattaaatgagtatttaatccttttaaattacattttgaaaatttaatggcaattacacacaaattttaatttaaaataatattaaggacttaatctgatttacagaaatgaaatgcaatgaagagattaagggctaacctccattactataaaattctctggctaccatctagcacaggagcaactggattgctttcagcagtcttgaagcactaaaatatcttaaaattcatatggagaaatagtatgtatctctacattaaatttagatttgatatttattctctgacagatcagacccagaatattaatttttatgtaattgaaccaaaaacatttagcaatccttcatttagtaatcttttgtataaatataaaaatctctgataagtgaaatgttttttcaaattatacttctatttttcacagctttataggtaattataattttcaaactttaaatatttcatgtgatttgatatatctgtacagaaagagtaagataaaaacatttaataagattaaatctaatttgcaaaaattggtatctgacatttgttgtgtgctcttgcaaagagtgcataggacatttctgcagcaatcaaaaaggtaaaatctttttaaactcagatttcaagtttcctctaatattccttctaatcctaatccctggaaatactttcaagttttgatttctagatgcaatgtgttttgttacatatacacatgtcttatccttaaacttttaaaaaacagtatgatcagattcagcatgatgatatcttctcagactctgtagaagtcctctgtgcaagattaatgtcgagattcctagtgccccatcgtgaaaaaccagttaaagatagtatacaactatgctttagtgggatttcctgcaggtttgggatcataaccatacaaaaaagtagctgttattacaaggatggctccaaggaaaaagacactggttggcacaaaatcttgaagccaaaaataggagatcaatgttgataatattatcgataaagaggttgcaaatccttttaaaatattatctgcatacttaataacagcagctattacaaggcctccaagtgcctgaagaacaactactatccaggtcagtcggttatatccctgaaaaaatccattctttgataccagttctccatcataaatgtatacacccattaatccaaatatacttccaaagaaaccaagctgaatatttcttatccacactgattgttttgtttcttttaagattttctcaaagtaaaccccagcaaagccacttgaaaaacatgctgtgagaactgccatgagtcctacaaattgagaaccagctgaaagttccttagaatcaagctgagaatctgagggccactgataagtagctgcatctagatttgatagtgccacatacagtaaattattctgaagagtatagatccctgatggaatagcaagtttaagtgtttccataggtttattaagaatttcatcatgtagtactcgattcagtgctcttagactacatttgctgtctttgtagaccaataaaatgcaggccattatcttcaaaagttcagcaacaaccactgctgtagaagatagataacgaggtccttcttcttttaaagttctggaataacgcattgttagaaccaaactggtagtctgaaagaccaaaattcccagggaaacgtattttaggttggcgaacattgttttatcttcatttgcctcccgcgcagctcgaccggctgagcccaccaccgggggccgcggttcagctccgccgggcgccccaggctgccgagtccgctgggtcctacgcgaccgctgacccgcagcgccgccggctcccgtcgccgtagccaccgccagctcggtgcagcccaggcgtttccgggttcccgcggtcccgtcccccaaatgctccggcttccgcctcggctctggcaaatgccgttcccggctcggctctggcagccccagctcggcacttggcagctctgtccctaaggcgacgcacctgggctgctctgctggcagcccctggttcctgcttcaccgtcgcgtggaggcctggggcactgctttctgctacacctctcctaggagcgcgaaacagatggagtgacactcgtcgagggcctctgcgggactgtctgtttgcagagggtgccaaggtgtccactgcgtaaggaagggcaaagtcctttggggcaaagaaccctgagaggaacggggagatggattttgaaagcaaacgaaccctctcctaaaagtgactgtcactgacctgaaaacaaccagattagctatggcaaaggctgccaaccaaccagtggtctgcaagaaggcttgttcttccacttcacccaccctgactgagatcttgagactgaaggaaacccaaagccgtaccaccaatgggcctagtgtcatcaaccgggagaggaaaaagaaaactgggcccagaggattgcagagttatgagggaccaaccccttcctggctgcatggatcacagcattaccttttaaaagtgttccagtagctgtgttggaaaccctctaaccacggcagcccattcaggtgatgaacaggctgaaatcagtacttcaggttcagctggattatcaaataagcgaataggattatctctttttgttaactcagggctgctataaattaagcctatgtctctttatattgcaaatgattaaaaccatgtccaagagagacatacttagaaaaaaagtgatattgaagaaaaataagtaactgtattagagtagaataactggttttaaaattttctgcaatacagtcttgagaaaattcctggatggtaaaatacatattagatcttaatacatgcccagttttttttgaaaccaaaatgtgcctgttagatgatgataacagcatgcctcgttttattgtgatttgctttattgctcttcacagacattgcttttgtttttttgttttttttttttacaaattgaaggtttgtggcaaccttgcctcaagcacatctattggtgccatttttccaacagcatgtgctcactttgtgtctctgtgtcacataatattcaataatttttgcaatatttaaatttgttcatcattattatatctggtatagtgctttgtgatcaatgatctttgatgttactatggtaattgttttggggtgctgatatggtttggctgtgtccccacccaaatctcaacttgaactgtatctcccagaattcccacgtgttgagggagagacctagggggagataattgaatcatgggggccagtctttcctgtgctattctcatgatagtgaataagtctcatgaaatccgatgggtttatctggggtttctgattttgcttcttcctcatttttctcttgctgcagccatgtaagcaagtacctttcacctcccgccatgattctgaggcctcccccgccatgtggaactgtaggtccaatta

SEQ ID NO: 15564 - RNA, 2953 nt, Homo sapiens
  source 1..2953: mol_type = other RNA
gctgggattacaggcatgagccactgtgcccagacagtaaaatacttcttatactcagtaagtaattctgtctatagttaataattaaattaaacccatattcaaattatagaaagcatttttgcccaccaaatcatcttaccatttctaatatactctctctctcttgaatcaacttattaaataactcatgtaatctgcatcctcagctccagtgttcattaaaaaggaaaaaaacccactattttaaagcaaaatggtggctccttctcagtagcttttttttttttcttttttttgagacagactctcactgtgtcgcccaggttggagtgcagtggcgtgatctccacttactgcaacctctgcctcccgggttcaagtgattctcctgcctcagtctcccgagtagctgggactacaggtgcgtgccaccacacccagctaatttttgtatttttggtagagacggggtttcaccatgttggtcaggatagtctcaatctcttgaccttgtgatccacctgcctcagcctcccaaactgctaggattacaggcgtgagccactgcgccaggccttctcagcagctcttgtgggaacacagaaagggaattcaaaatttggctacctctcccactcatgtgatcagggaagaataggcttatgagagacctaaaaaaatcttccgagcagccttggatttaaagtcatagcgctgtttaaaataaagtaatatggcaatctggaatgtctccaagaaaagtcattttgttctgtcactgacatctgtactatttgtttgaatgttgtttttgtaaacagttgtagattaaagaagtttttacagatcaatgagtaaaatgttcatttaataactttctaactgtatacagtatatgcttgatagttcaaaattctccaaatgtagatattatacaataattattttaaattattaaatgagtatttaatccttttaaattacattttgaaaatttaatggcaattacacacaaattttaatttaaaataatattaaggacttaatctgatttacagaaatgaaatgcaatgaagagattaagggctaacctccattactataaaattctctggctaccatctagcacaggagcaactggattgctttcagcagtcttgaagcactaaaatatcttaaaattcatatggagaaatagtatgtatctctacattaaatttagatttgatatttattctctgacagatcagacccagaatattaatttttatgtaattgaaccaaaaacatttagcaatccttcatttagtaatcttttgtataaatataaaaatctctgataagtgaaatgttttttcaaattatacttctatttttcacagctttataggtaattataattttcaaactttaaatatttcatgtgatttgatatatctgtacagaaagagtaagataaaaacatttaataagattaaatctaatttgcaaaaattggtatctgacatttgttgtgtgctcttgcaaagagtgcataggacatttctgcagcaatcaaaaaggtaaaatctttttaaactcagatttcaagtttcctctaatattccttctaatcctaatccctggaaatactttcaagttttgatttctagatgcaatgtgttttgttacatatacacatgtcttatccttaaacttttaaaaaacagtatgatcagattcagcatgatgatatcttctcagactctgtagaagtcctctgtgcaagattaatgtcgagattcctagtgccccatcgtgaaaaaccagttaaagatagtatacaactatgctttagtgggatttcctgcaggtttgggatcataaccatacaaaaaagtagctgttattacaaggatggctccaaggaaaaagacactggttggcacaaaatcttgaagccaaaaataggagatcaatgttgataatattatcgataaagaggttgcaaatccttttaaaatattatctgcatacttaataacagcagctattacaaggcctccaagtgcctgaagaacaactactatccaggtcagtcggttatatccctgaaaaaatccattctttgataccagttctccatcataaatgtatacacccattaatccaaatatacttccaaagaaaccaagctgaatatttcttatccacactgattgttttgtttcttttaagattttctcaaagtaaaccccagcaaagccacttgaaaaacatgctgtgagaactgccatgagtcctacaaattgagaaccagctgaaagttccttagaatcaagctgagaatctgagggccactgtacaaaagcaactcctgtcatcaaaattactagggacagccactggtatacacccaattttttactaagcatagacacagaaaataatgctgttgtaagaatttttaactgatacgtgacctgataagtagctgcatctagatttgatagtgccacatacagtaaattattctgaagagtatagatccctgatggaatagcaagtttaagtgtttccataggtttattaagaatttcatcatgtagtactcgattcagtgctcttagactacatttgctgtctttgtagaccaataaaatgcaggccattatcttcaaaagttcagcaacaaccactgctgtagaagatagataacgaggtccttcttcttttaaagttctggaataacgcattgttagaaccaaactggtagtctgaaagaccaaaattcccagggaaacgtattttaggttggcgaacattgttttatcttcatttgccaagggcagcctttccatttctttaagttcctgcggcttcttgagctccaggtgctggtcgggtgcatctgtgcctaccacagggctcaacaccgagcgagagctcatgggatgttcactgaaggaat

SEQ ID NO: 15565 - RNA, 2992 nt, Homo sapiens
  source 1..2992: mol_type = other RNA
gctgggattacaggcatgagccactgtgcccagacagtaaaatacttcttatactcagtaagtaattctgtctatagttaataattaaattaaacccatattcaaattatagaaagcatttttgcccaccaaatcatcttaccatttctaatatactctctctctcttgaatcaacttattaaataactcatgtaatctgcatcctcagctccagtgttcattaaaaaggaaaaaaacccactattttaaagcaaaatggtggctccttctcagtagcttttttttttttcttttttttgagacagactctcactgtgtcgcccaggttggagtgcagtggcgtgatctccacttactgcaacctctgcctcccgggttcaagtgattctcctgcctcagtctcccgagtagctgggactacaggtgcgtgccaccacacccagctaatttttgtatttttggtagagacggggtttcaccatgttggtcaggatagtctcaatctcttgaccttgtgatccacctgcctcagcctcccaaactgctaggattacaggcgtgagccactgcgccaggccttctcagcagctcttgtgggaacacagaaagggaattcaaaatttggctacctctcccactcatgtgatcagggaagaataggcttatgagagacctaaaaaaatcttccgagcagccttggatttaaagtcatagcgctgtttaaaataaagtaatatggcaatctggaatgtctccaagaaaagtcattttgttctgtcactgacatctgtactatttgtttgaatgttgtttttgtaaacagttgtagattaaagaagtttttacagatcaatgagtaaaatgttcatttaataactttctaactgtatacagtatatgcttgatagttcaaaattctccaaatgtagatattatacaataattattttaaattattaaatgagtatttaatccttttaaattacattttgaaaatttaatggcaattacacacaaattttaatttaaaataatattaaggacttaatctgatttacagaaatgaaatgcaatgaagagattaagggctaacctccattactataaaattctctggctaccatctagcacaggagcaactggattgctttcagcagtcttgaagcactaaaatatcttaaaattcatatggagaaatagtatgtatctctacattaaatttagatttgatatttattctctgacagatcagacccagaatattaatttttatgtaattgaaccaaaaacatttagcaatccttcatttagtaatcttttgtataaatataaaaatctctgataagtgaaatgttttttcaaattatacttctatttttcacagctttataggtaattataattttcaaactttaaatatttcatgtgatttgatatatctgtacagaaagagtaagataaaaacatttaataagattaaatctaatttgcaaaaattggtatctgacatttgttgtgtgctcttgcaaagagtgcataggacatttctgcagcaatcaaaaaggtaaaatctttttaaactcagatttcaagtttcctctaatattccttctaatcctaatccctggaaatactttcaagttttgatttctagatgcaatgtgttttgttacatatacacatgtcttatccttaaacttttaaaaaacagtatgatcagattcagcatgatgatatcttctcagactctgtagaagtcctctgtgcaagattaatgtcgagattcctagtgccccatcgtgaaaaaccagttaaagatagtatacaactatgctttagtgggatttcctgcaggtttgggatcataaccatacaaaaaagtagctgttattacaaggatggctccaaggaaaaagacactggttggcacaaaatcttgaagccaaaaataggagatcaatgttgataatattatcgataaagaggttgcaaatccttttaaaatattatctgcatacttaataacagcagctattacaaggcctccaagtgcctgaagaacaactactatccaggtcagtcggttatatccctgaaaaaatccattctttgataccagttctccatcataaatgtatacacccattaatccaaatatacttccaaagaaaccaagctgaatatttcttatccacactgattgttttgtttcttttaagattttctcaaagtaaaccccagcaaagccacttgaaaaacatgctgtgagaactgccatgagtcctacaaattgagaaccagctgaaagttccttagaatcaagctgagaatctgagggccactgtacaaaagcaactcctgtcatcaaaattactagggacagccactggtatacacccaattttttactaagcatagacacagaaaataatgctgttgtaagaatttttaactgatacgtgacctgataagtagctgcatctagatttgatagtgccacatacagtaaattattctgaagagtatagatccctgatggaatagcaagtttaagtgtttccataggtttattaagaatttcatcatgtagtactcgattcagtgctcttagactacatttgctgtctttgtagaccaataaaatgcaggccattatcttcaaaagttcagcaacaaccactgctgtagaagatagataacgaggtccttcttcttttaaagttctggaataacgcattgttagaaccaaactggtagtctgaaagaccaaaattcccagggaaacgtattttaggttggcgaacattgttttatcttcatttgcctcccgcgcagctcgaccggctgagcccaccaccgggggccgcggttcagctccgccgggcgccccaggctgccgagtccgctgggtcctacgcgaccgctgacccgcagcgccgccggctcccgtcgccgtagccaccgccagctcggtgcagcccaggcgtttcc

SEQ ID NO: 15566 - RNA, 3116 nt, Homo sapiens
  source 1..3116: mol_type = other RNA
gctgggattacaggcatgagccactgtgcccagacagtaaaatacttcttatactcagtaagtaattctgtctatagttaataattaaattaaacccatattcaaattatagaaagcatttttgcccaccaaatcatcttaccatttctaatatactctctctctcttgaatcaacttattaaataactcatgtaatctgcatcctcagctccagtgttcattaaaaaggaaaaaaacccactattttaaagcaaaatggtggctccttctcagtagcttttttttttttcttttttttgagacagactctcactgtgtcgcccaggttggagtgcagtggcgtgatctccacttactgcaacctctgcctcccgggttcaagtgattctcctgcctcagtctcccgagtagctgggactacaggtgcgtgccaccacacccagctaatttttgtatttttggtagagacggggtttcaccatgttggtcaggatagtctcaatctcttgaccttgtgatccacctgcctcagcctcccaaactgctaggattacaggcgtgagccactgcgccaggccttctcagcagctcttgtgggaacacagaaagggaattcaaaatttggctacctctcccactcatgtgatcagggaagaataggcttatgagagacctaaaaaaatcttccgagcagccttggatttaaagtcatagcgctgtttaaaataaagtaatatggcaatctggaatgtctccaagaaaagtcattttgttctgtcactgacatctgtactatttgtttgaatgttgtttttgtaaacagttgtagattaaagaagtttttacagatcaatgagtaaaatgttcatttaataactttctaactgtatacagtatatgcttgatagttcaaaattctccaaatgtagatattatacaataattattttaaattattaaatgagtatttaatccttttaaattacattttgaaaatttaatggcaattacacacaaattttaatttaaaataatattaaggacttaatctgatttacagaaatgaaatgcaatgaagagattaagggctaacctccattactataaaattctctggctaccatctagcacaggagcaactggattgctttcagcagtcttgaagcactaaaatatcttaaaattcatatggagaaatagtatgtatctctacattaaatttagatttgatatttattctctgacagatcagacccagaatattaatttttatgtaattgaaccaaaaacatttagcaatccttcatttagtaatcttttgtataaatataaaaatctctgataagtgaaatgttttttcaaattatacttctatttttcacagctttataggtaattataattttcaaactttaaatatttcatgtgatttgatatatctgtacagaaagagtaagataaaaacatttaataagattaaatctaatttgcaaaaattggtatctgacatttgttgtgtgctcttgcaaagagtgcataggacatttctgcagcaatcaaaaaggtaaaatctttttaaactcagatttcaagtttcctctaatattccttctaatcctaatccctggaaatactttcaagttttgatttctagatgcaatgtgttttgttacatatacacatgtcttatccttaaacttttaaaaaacagtatgatcagattcagcatgatgatatcttctcagactctgtagaagtcctctgtgcaagattaatgtcgagattcctagtgccccatcgtgaaaaaccagttaaagatagtatacaactatgctttagtgggatttcctgcaggtttgggatcataaccatacaaaaaagtagctgttattacaaggatggctccaaggaaaaagacactggttggcacaaaatcttgaagccaaaaataggagatcaatgttgataatattatcgataaagaggttgcaaatccttttaaaatattatctgcatacttaataacagcagctattacaaggcctccaagtgcctgaagaacaactactatccaggtcagtcggttatatccctgaaaaaatccattctttgataccagttctccatcataaatgtatacacccattaatccaaatatacttccaaagaaaccaagctgaatatttcttatccacactgattgttttgtttcttttaagattttctcaaagtaaaccccagcaaagccacttgaaaaacatgctgtgagaactgccatgagtcctacaaattgagaaccagctgaaagttccttagaatcaagctgagaatctgagggccactgtacaaaagcaactcctgtcatcaaaattactagggacagccactggtatacacccaattttttactaagcatagacacagaaaataatgctgttgtaagaatttttaactgatacgtgacctgataagtagctgcatctagatttgatagtgccacatacagtaaattattctgaagagtatagatccctgatggaatagcaagtttaagtgtttccataggtttattaagaatttcatcatgtagtactcgattcagtgctcttagactacatttgctgtctttgtagaccaataaaatgcaggccattatcttcaaaagttcagcaacaaccactgctgtagaagatagataacgaggtccttcttcttttaaagttctggaataacgcattgttagaaccaaactggtagtctgaaagaccaaaattcccagggaaacgtattttaggttggcgaacattgttttatcttcatttgcttgggaggctaaggtgggagatcacttgagccagggaggtggaagttgcagtgagctgagattgcgcctctgtactccagccaaggtgacagtgagacccaagggcagcctttccatttctttaagttcctgcggcttcttgagctccaggtgctggtcgggtgcatctgtgcctaccacagggctcaacaccgagcgagagctcatgggatgttcactgaaggaatgacgggccccagccgggcccacccgtcactagctccgcacgcaccaggcgctgaggcacacact

SEQ ID NO: 15567 - RNA, 4686 nt, Homo sapiens
  source 1..4686: mol_type = other RNA
gctgggattacaggcatgagccactgtgcccagacagtaaaatacttcttatactcagtaagtaattctgtctatagttaataattaaattaaacccatattcaaattatagaaagcatttttgcccaccaaatcatcttaccatttctaatatactctctctctcttgaatcaacttattaaataactcatgtaatctgcatcctcagctccagtgttcattaaaaaggaaaaaaacccactattttaaagcaaaatggtggctccttctcagtagcttttttttttttcttttttttgagacagactctcactgtgtcgcccaggttggagtgcagtggcgtgatctccacttactgcaacctctgcctcccgggttcaagtgattctcctgcctcagtctcccgagtagctgggactacaggtgcgtgccaccacacccagctaatttttgtatttttggtagagacggggtttcaccatgttggtcaggatagtctcaatctcttgaccttgtgatccacctgcctcagcctcccaaactgctaggattacaggcgtgagccactgcgccaggccttctcagcagctcttgtgggaacacagaaagggaattcaaaatttggctacctctcccactcatgtgatcagggaagaataggcttatgagagacctaaaaaaatcttccgagcagccttggatttaaagtcatagcgctgtttaaaataaagtaatatggcaatctggaatgtctccaagaaaagtcattttgttctgtcactgacatctgtactatttgtttgaatgttgtttttgtaaacagttgtagattaaagaagtttttacagatcaatgagtaaaatgttcatttaataactttctaactgtatacagtatatgcttgatagttcaaaattctccaaatgtagatattatacaataattattttaaattattaaatgagtatttaatccttttaaattacattttgaaaatttaatggcaattacacacaaattttaatttaaaataatattaaggacttaatctgatttacagaaatgaaatgcaatgaagagattaagggctaacctccattactataaaattctctggctaccatctagcacaggagcaactggattgctttcagcagtcttgaagcactaaaatatcttaaaattcatatggagaaatagtatgtatctctacattaaatttagatttgatatttattctctgacagatcagacccagaatattaatttttatgtaattgaaccaaaaacatttagcaatccttcatttagtaatcttttgtataaatataaaaatctctgataagtgaaatgttttttcaaattatacttctatttttcacagctttataggtaattataattttcaaactttaaatatttcatgtgatttgatatatctgtacagaaagagtaagataaaaacatttaataagattaaatctaatttgcaaaaattggtatctgacatttgttgtgtgctcttgcaaagagtgcataggacatttctgcagcaatcaaaaaggtaaaatctttttaaactcagatttcaagtttcctctaatattccttctaatcctaatccctggaaatactttcaagttttgatttctagatgcaatgtgttttgttacatatacacatgtcttatccttaaacttttaaaaaacagtatgatcagattcagcatgatgatatcttctcagactctgtagaagtcctctgtgcaagattaatgtcgagattcctagtgccccatcgtgaaaaaccagttaaagatagtatacaactatgctttagtgggatttcctgcaggtttgggatcataaccatacaaaaaagtagctgttattacaaggatggctccaaggaaaaagacactggttggcacaaaatcttgaagccaaaaataggagatcaatgttgataatattatcgataaagaggttgcaaatccttttaaaatattatctgcatacttaataacagcagctattacaaggcctccaagtgcctgaagaacaactactatccaggtcagtcggttatatccctgaaaaaatccattctttgataccagttctccatcataaatgtatacacccattaatccaaatatacttccaaagaaaccaagctgaatatttcttatccacactgattgttttgtttcttttaagattttctcaaagtaaaccccagcaaagccacttgaaaaacatgctgtgagaactgccatgagtcctacaaattgagaaccagctgaaagttccttagaatcaagctgagaatctgagggccactgtacaaaagcaactcctgtcatcaaaattactagggacagccactggtatacacccaattttttactaagcatagacacagaaaataatgctgttgtaagaatttttaactgatacgtgacctgataagtagctgcatctagatttgatagtgccacatacagtaaattattctgaagagtatagatccctgatggaatagcaagtttaagtgtttccataggtttattaagaatttcatcatgtagtactcgattcagtgctcttagactacatttgctgtctttgtagaccaataaaatgcaggccattatcttcaaaagttcagcaacaaccactgctgtagaagatagataacgaggtccttcttcttttaaagttctggaataacgcattgttagaaccaaactggtagtctgaaagaccaaaattcccagggaaacgtattttaggttggcgaacattgttttatcttcatttgcttgggaggctaaggtgggagatcacttgagccagggaggtggaagttgcagtgagctgagattgcgcctctgtactccagccaaggtgacagtgagaccctcccgcgcagctcgaccggctgagcccaccaccgggggccgcggttcagctccgccgggcgccccaggctgccgagtccgctgggtcctacgcgaccgctgacccgcagcgccgccggctcccgtcgccgtagccaccgccagctcggtgcagcccaggcgtttccgggttcccgcggtcccgtcccccaaatgctccggcttccgcctcggctctggcaaatgccgttcccggctcggctctggcagccccagctcggcacttggcagctctgtccctaaggcgacgcacctgggctgctctgctggcagcccctggttcctgcttcaccgtcgcgtggaggcctggggcactgctttctgctacacctctcctaggagcgcgaaacagatggagtgacactcgtcgagggcctctgcgggactgtctgtttgcagagggtgccaaggtgtccactgcgtaaggaagggcaaagtcctttggggcaaagaaccctgagaggaacggggagatggattttgaaagcaaacgaaccctctcctaaaagtgactgtcactgacctgaaaacaaccagattagctatggcaaaggctgccaaccaaccagtggtctgcaagaaggcttgttcttccacttcacccaccctgactgagatcttgagactgaaggaaacccaaagccgtaccaccaatgggcctagtgtcatcaaccgggagaggaaaaagaaaactgggcccagaggattgcagagttatgagggaccaaccccttcctggctgcatggatcacagcattaccttttaaaagtgttccagtagctgtgttggaaaccctctaaccacggcagcccattcaggtgatgaacaggctgaaatcagtacttcaggttcagctggattatcaaataagcgaataggattatctctttttgttaactcagggctgctataaattaagcctatgtctctttatattgcaaatgattaaaaccatgtccaagagagacatacttagaaaaaaagtgatattgaagaaaaataagtaactgtattagagtagaataactggttttaaaattttctgcaatacagtcttgagaaaattcctggatggtaaaatacatattagatcttaatacatgcccagttttttttgaaaccaaaatgtgcctgttagatgatgataacagcatgcctcgttttattgtgatttgctttattgctcttcacagacattgcttttgtttttttgttttttttttttacaaattgaaggtttgtggcaaccttgcctcaagcacatctattggtgccatttttccaacagcatgtgctcactttgtgtctctgtgtcacataatattcaataatttttgcaatatttaaatttgttcatcattattatatctggtatagtgctttgtgatcaatgatctttgatgttactatggtaattgttttggggtgctgatatggtttggctgtgtccccacccaaatctcaacttgaactgtatctcccagaattcccacgtgttgagggagagacctagggggagataattgaatcatgggggccagtctttcctgtgctattctcatgatagtgaataagtctcatgaaatccgatgggtttatctggggtttctgattttgcttcttcctcatttttctcttgctgcagccatgtaagcaagtacctttcacctcccgccatgattctgaggcctcccccgccatgtggaactgtaggtccaatta

SEQ ID NO: 15568 - RNA, 3877 nt, Homo sapiens
  source 1..3877: mol_type = other RNA
gctgggattacaggcatgagccactgtgcccagcactgaccatttaaaagagcgtctttgcttacttccttcttagcagtgtttaagggcaaccatcgcagattgagctcagcctaatttcaaatttgcatgacatagagtgttttatggaggggctggcctttcctttctatcttttgctgagtcttagagaatgctcatgaatgttccttctggtctatggtttccccttcacttaaaaataagaattaatactgcaaaatctgaaatctcattcactccttcatgagcaggtcctgatataaatacatccagaattcagtccatctattatgataacattgtagcaaccccctgtatccacatagattattgtcttgaacatatgacattctcataccacatgattctgcagtaaatctaacagcagttctaaataaggccaaaaaggagagtgctttgtcaaaactaaaagcaccatccacccaaatgtgaagtgtcatcacgatggcatccattcccctaagtttctttcagcaatgtgacttgagaaccaaccctcaatgaaaactcgaatctcctaaccagttatataaattttaaatctaggagctagttcttctttcatggattttggattctctttgtgatgttggtttgtctcaatttagtcccatttcttgctttgtaaacctgcgattatatgcctcctagtaaaccacatgatatgatcagcgctgctttcatagtctctgaactgttgcttaaaaagaacagatataattgcatggtaagtcattcaggttgctctttactggtgaaatgaagagaaacctgggtgtcctctgatgtctgtctatacaccccacctccctgattcacagaaccattttccggtttcacttcttgcttcttttatcttgtgcatttttagcacctgttgtgacaagcctgggtgactcgatctaaaaaatgaaatgacttacaattactgtaagaatgaattacagatacatgatgtatgcacaactctgtatagaaatgaaaacaaaaataacttcacctcactctaattcataggctaccatgttattgacccttatttacctaacttttgcttaagcaggaaagatccctctgcctagatatcccctgggcttggcgccctcactcctccaccccagcccttatgcatttggcagtagtaatggcccctgcagggaatgttgtccaagaagtctagatgatagagatgaagaaggcacatcacttcacagagtttatgccaagtcaccgccagaagcgcagtgttacaatttacttaagccaagactgctacaaaaaactgatgcaaatggaagctattcaaaatcctttgccttgtgcattcaagttgaggctcccttttgaatcctatctctgagtctacatctgctgggtaaattcctgaacgatgacttgagctgtgacagcttttgtagcattgctgtggtccaaccacaactctgtaagataaactacctaagctggttgttggacttcctctaaaatgtcattctaattatagaaacacctttctttcctgattttatacagattctaatcaccttaactgcttctcttcagccatgaatgaaagcgaaagattaagtcacttttagaagccttcttgggcaattatagattaattcatttctcgctcattgaagggactcaatcctagaacaacagtctggaatacatgtgtatgtatgcccctttgtctctgacctgctcatcattggccatcaatgccctgggaaggagggaccctaggaaggcctgaggggctgcacctgatgtgcaggtcatgtgcacagaccccacaggttcaggctcagtgttgaaattccctatgtcattaactcccttgtaggaaggatgaaagggtctagatcagatttaagtcagacataggctatttgaggcgcctgtgggaatggcaaatcactccagactcctcagaagcaaaggccaagcaggcctgagagctagtgaaactccagggagaggagcaagaccaggatctgcgctttctcagcttcccaaagctgtctgtctcggaactaacaaatgaggctgactcttcagagttctaggccaagggatccggacttgacactcaagtttctgccatgaagcaaaagacagagctagcctggaaagagcagctctgtatcactccggctgtgaagtgctaaaactcgacatctccctgaggaaacaggagagaagaaaggatggagagaaaaaaagagaggaaggagctggcattaatggaccagcaagggaaggagaagggagcaggaaaagcggtagttcacgtagggtaaattagatgaaggggaacaaacagcgaaaggtcagagggctctgcacttaaaataaggaagcttgtgaagataagtaaatgttgcctgagatatctgaagtagggttcctctttggctgacaagccttaatctgcactctggaaacagcttgtatgaggaggaggacggcagacaaggaggaatgagggaggaattcttacaggaaccatctggctgagtcacttttagggctgttcaaagctacccaactgttgacatttcctggaaattctttaatgccaacaattgtgttaaatgagcaacatccttaagaccccgagtgcaccttggatcccctcgtcctttcttgttgcgtttgcgatttgcaaatcccctgaacctgaagtcttcaaggattcagcatctgccatttcaccatgtgttagtcccctccctgggccccttcaaacacactctccactcagaaatctaccatttagcctttatttatttatttatttatttatttttgacgcacgcacaaggcttctcactcctcctcagctttcaaagaatccacccactaggctgtcacttcaatctgctgtctcctcctgcagcacagaatttctgaagaaagtccccaggtgaaccagcctggccagcagaaatggatgctcacccactccatctagcccctggcctctgctctcctggactccctggctcagtcctcagatcagttccggaacttctctccttaggtttcctgtaacatccgggtttctcccttacttgcttaaaacaacctcttgctttcattcatccattcattcactctgaggccatctgaggaaagcttccttacctgctttcctgatgacctaatatatgctgtacccacctacttcctcttccttgaatggggaaaccaagtcacagggaaagatacatctctcccttctaatgctggatctcattccttacaagcctgctctcattctccacctccaatctctctgtgtccattcttctcttcttttcatccgtcagttatgccagtggctcccagcctggagtatgaatctgggggcaggggtgtctctgaaagttctggaggctgggaagtccaacagcatggcactggcatctggtgagagtcttcttgctgtggcataaccctccccgtccctgctaaagcctccttgtactttcttccacttgcatttccatatccctgacccatctacagggctcggaaaaagccttttcacacgtgatatgttcagataagttaaatcccctgaaattctgcgtgacgtggtgtatctgtgccatttagtgtcgttccattgatccacagacttgggagcagttcagatctgagggaacaaaagctggtccaaggacatcattgtcaaatcttcaacccacaggcaggctctcccagcacctcgggaactctgtgtcacagcagtccatggaagtattgccctggctacaggcagacacttcacaaagaggat

SEQ ID NO: 15569 - RNA, 2265 nt, Homo sapiens
  source 1..2265: mol_type = other RNA
gctgggattacaggcatgagccactgtgcccagccaacacaacatacttttaatgaaaaataactacatttttccaaaccaaaaagaaagtgaaaacagtggtattgttttgtattttttgcaaatctcttcaatgtctggtttaatattctggtttaattcccatatctgcttctatactcaacctgtttcaacatcacatgtcacaaacagccaggcgcagtggctcacacctataatcccagcactttgggaggtgaaggcgggaggatcacttgaggccaggagttggaagaccagtctgggcaacatagcaagacccctctgtcagtataaaaaacaaaataaaaaaacacatgtcatgtagcctctggaaaatcccactgtacactcatgaaagacaaataatatctttttttttttttttgagacagtgtcttgctccatcacccaggctggagtgcagtggtgagatttcagctcactgcaatctctgcctcccggattcaagcaattctcctgcctcagcctcctcctgagtagctgggattacaggcatgcatcaccacacccaggtaatttttgtatttttagtagagactgggtttcaccatgttggccaggctggtctgaaactcctgacctcattatccatttgccttggcctcccaaagtgctgagattataggcgtgagccaccgtgcccagctgacaaataacatcttaatattaccgtgaacctagtgtagactttatggatacttcaaaaggaccgcactttggaaaccacagagttaaacaatatcaagtctcattggcttcatgcaataaaaatgtactccaatgaagactggccagcttcccatggagagctggctttttccatcatgctgtaaattataccatctggaatgcgtggtttccaagtttactgagagagagaagggggctggtgaatcaggtgggatgcttttaagggtagggcctgagccaggcacactggctcatgcctatatgacatcagctattagggaggctgaggtgggaggattgtttgagcacaggaggttgaggctgcagtgagtcatgatcacagcactgcactccagcctgggtgacagaacaagactcagacctttaaataaaaaaaagactagggcctagaggtggggcatgtcactggaaatgtcatcttcctgtgtgtccaggaagagaattgggtgtggtgaacacttagcatctgctccacccctggggtgatcgtggcgctcacatgatcctgtgaccggaagcctccacagggtcacttcatgaacatttctcatgtttctgcagcattttcaaacagttgccctgttagtgacagcagttataacaggtgactttgacttcgagcatttgtcccattcaaattaatttttctattttaattataaaagtaatacatgttcacacacacaaagcatcatttcaatgatcagaaggacaaaagagaaagataaacattacaccccatggaacctccttgaactgtgtcaccacccgcgagaagcatagtgaattctctcaaaaagtttctttgcatctctaagcttacatctacatctattttttggaatgcagttggggtcatattatgcatactgttctataaatccggaaggaggggcattaagtagacaagatgatatgcagaagcagatggaaggtagaaaaactcctctgcatgaattcagggctccctctggcttcaaagacggtttcctttgccaacaccaaggagtaggctccagcctgggttgctgagaggacatgggaggactcctgggacttcttcagctgttacccagccttgtgctgatgagaccaggcatagacagtcctgacgacacagggcggaagggagcagccattagtgctaatgaggcaggcggcctgaaagctttgtactctgcagtggctcgcccacccagggaacagttcgttctgtttccttggcttccaggaaccctaggcagaaaggggtttggggacaggagcaggagtgggcggtcttggagaaacctcaatcggacctcagtttccctctggggaggaggctggcccagcagtctggaaactttccaagcttgagaagggctcgctcccttctttaccccgcccgccctgcagcgtcaagtgcagcaaaccggggaaagctagagaaggcccagtcaaatccctgcggccacaggcgccaccaagcggccggcctcaaacttcctc

SEQ ID NO: 15570 - RNA, 1862 nt, Homo sapiens
  source 1..1862: mol_type = other RNA
gctgggattacaggcatgagccactgtgcccagccaacacaacatacttttaatgaaaaataactacatttttccaaaccaaaaagaaagtgaaaacagtggtattgttttgtattttttgcaaatctcttcaatgtctggtttaatattctggtttaattcccatatctgcttctatactcaacctgtttcaacatcacatgtcacaaacagccaggcgcagtggctcacacctataatcccagcactttgggaggtgaaggcgggaggatcacttgaggccaggagttggaagaccagtctgggcaacatagcaagacccctctgtcagtataaaaaacaaaataaaaaaacacatgtcatgtagcctctggaaaatcccactgtacactcatgaaagacaaataatatctttttttttttttttgagacagtgtcttgctccatcacccaggctggagtgcagtggtgagatttcagctcactgcaatctctgcctcccggattcaagcaattctcctgcctcagcctcctcctgagtagctgggattacaggcatgcatcaccacacccaggtaatttttgtatttttagtagagactgggtttcaccatgttggccaggctggtctgaaactcctgacctcattatccatttgccttggcctcccaaagtgctgagattataggcgtgagccaccgtgcccagctgacaaataacatcttaatattaccgtgaacctagtgtagactttatggatacttcaaaaggaccgcactttggaaaccacagagttaaacaatatcaagtctcattggcttcatgcaataaaaatgtactccaatgaagactggccagcttcccatggagagctggctttttccatcatgctgtaaattataccatctggaatgcgtggtttccaagtttactgagagagagaagggggctggtgaatcaggtgggatgcttttaagggtagggcctgagccaggcacactggctcatgcctatatgacatcagctattagggaggctgaggtgggaggattgtttgagcacaggaggttgaggctgcagtgagtcatgatcacagcactgcactccagcctgggtgacagaacaagactcagacctttaaataaaaaaaagactagggcctagaggtggggcatgtcactggaaatgtcatcttcctgtgtgtccaggaagagaattgggtgtggtgaacacttagcatctgctccacccctggggtgatcgtggcgctcacatgatcctgtgaccggaagcctccacagggtcacttcatgaacatttctcatgtttctgcagcattttcaaacagttgcccttcaaagacggtttcctttgccaacaccaaggagtaggctccagcctgggttgctgagaggacatgggaggactcctgggacttcttcagctgttacccagccttgtgctgatgagaccaggcatagacagtcctgacgacacagggcggaagggagcagccattagtgctaatgaggcaggcggcctgaaagctttgtactctgcagtggctcgcccacccagggaacagttcgttctgtttccttggcttccaggaaccctaggcagaaaggggtttggggacaggagcaggagtgggcggtcttggagaaacctcaatcggacctcagtttccctctggggaggaggctggcccagcagtctggaaactttccaagcttgagaagggctcgctcccttctttaccccgcccgccctgcagcgtcaagtgcagcaaaccggggaaagctagagaaggcccagtcaaatccctgcggccacaggcgccaccaagcggccggcctcaa

SEQ ID NO: 15571 - RNA, 10042 nt, Homo sapiens
  source 1..10042: mol_type = other RNA
gctgggattacaggcatgagccactgtgcccagccaactctttacattttgaaacaatgtgttctttctgtaatcccaaagactcaaatacaatgaagtatgtactttcacctcaaaatgtgataaacaactaaattgggatgcaacctaggcagtaggctggattctctcacttgctaaacaacctggtctcaacttcagtctcagatttatgttgtaaaacatacacctgtgttaaaggtcatggaggaggagtggggcagcgcttagcatcagaatcaaatgtgataaacctaaagagacgagtcttttcatcttgttactctgcacagttttcatttggcctctagccacttagaccagcaactcagttttcaacacgtggtagggcaaactgtttggcatgttcacttatagaggcttgataaagtgtttccggaatatttttaaaatggagcagcattgtgcatttgttagaatgaatatttgacttaaaactgtactactgtatagattacatcaaactggaatagcctgaattctgttgacaagaaaatggtagttctagccttaaggctttgacccagtaagaactttcaatgacatgaaagctgtatggtgtttttttttttttttttttttttttttttttttttgagacggagtctcgctctgtcaccaggctggagcgtggtggtgcgatcttggctcactgcagcctccacctcccaggttcaagtgattctcctgcctcagcctcccgagtagctgggattacaggcacgtgccaccacgctcagctaatttttgtacttttagtagagattgggtttcaccatgttggccaggatggcctcattctctgtcctgatccgcccatcttggcctcccaaagtgctggagttacaggcgtgagccactctgcccagcctgtgtggtgtatttttaacacttctgtttttagaatatgcaagaaacacatggggatggttttatttttataattggttaaaaaagtttctcaaagtgaagtttaggagtgagttttagtgttttgtaatttgaagaaaagtgtcttaaaattcaaagataccaatggaaagataaaagtttgggttttagaggaatacatatttcatttttaaaattcataatttgcttcatactaagaatatgaagaatcctttacacttaatggttttgtacagcaaagtttaaaaataatttacattaaatggcaagtatgacttggatcaatagctcttcagttaatgagaaatgaagcaattttacttgaaagtctagcccatttcagatgttcagagcatatattttctttttagaagtttgtcttcaagtactgagaactaatgcttctaatccatggcaatatcaagagagcgatgtataataaatatataagtatagtgtcagtacaaaccttgcaaaataaatttaaacgccaactcaatctacttttgctttaaaaaattgttaggtttcttgttaagacattgcaattcagtagatattaaattatacgtcattctaaattcattttgaaaaccaaaaatgagtaatctaatctatgattaagcaataaccttttttaaagcaaccctattaactgaataggcaataaccttaaaaaaaacccaatattatttctatatgtaaaaaaatcctaaagaggagtgcactgtggtacacaatacaggaactaaattgaattttaatgactcttatgttataggacatatttacacttgaaatgccccaaagcttctaattctaagcttctaattctcggccataaaatgtatggctaaacttcctttcctgttttcagatctttgtgctccttgttcccagttctcttctcttagttgtgttggcaaattaaggtccttgggccaaatctagcctgccacctgtttttgtatggcccctgaattaagaatagtttttaagtttttaaatggttgaaaaaaagtcaaaacaagagtatttgtgacatgtgaaaaatatatgaaattccaatttcagtgtccataaataaagttttattggaatacagccacgttcgttcatgtatgtgttgtctatggctgcttttgcactacaatggcagaattgggtggttgcaacatattttatggcccccagccctaaaatatttactgtttggccctttacagacaagcttgctgacccttgctctaagtcaattcgtgacgatttttccaactgctgacatttataaaatggcagtcccctgggcttcattcatcagtaaattggttggtggcaactagccctgtgccattttgcttctcctcagcatggatctcacatgtgtgaaggcttcagttcagaaatcatcaatttccagtttaagtctgatgaaaataattatattttttccaccatgttcactctttaacttcttgcttaaagatcttcacctgggttaaacatgctgcccttagtcactgtcggtaatccattgtgtcactggaggacaagccacccacaggtttctcctccttggtttggatactttctgaggtcaagagctgagaaggtgatgtaagtcctcggggctgtttagttgacttggtgagcttcttgagttcacttgcgaaagaaatgcctttctttttatcttctcgagatgcctgcacctgctcctttagcttaaggatgaattttcctgcacctttccacttgctttgggcttgaaacacacactcctgatccagaaggacccgctgagaggactttggtgtggtagtcttcttgttggtagtgtctttcaccacctcttccaaaagcacatagtcgcttggattggggttgctcaggatgctgtaggaatatttggctttgcataaggtctgctgaatgacatcctgtgcagtgctgacgcggggtgctttgatgactgttcgaggttgctctggagaaacatcatgcacttggacaaagaaactctcctcctctgagctcaagatcacctctttgtcatcttgaacaatgtttttctcttctaggttttcctgctgggtttttaagacaatcctgcccatgtatccctcttctggaaaccagctgcttaaaatttgcatgatctcctcttctggaccaatggctctctggaatggttgtttcctacattcattcttttctttagatataaaatatttttcttccatcaaaaaatagtctgtggtaacaggtttgatgtcttgttcatttgtcagaatttgctgcagaagctgctttgccttggtgcctccattaatagtgaaaacggtaaagggctctggccctgggaccccatgcaccgtgactctgtgagtctgcaaacattttctttcttctgtattaaacatcgaagaggctgacatggtattgccagaggaattttcttccatccttctgctgttaatgaataaactagaaatctccaagacttcattgtgaaggtttcgcagctgaagatgtcgatatcctcgttttaaagctttcagtggaatgattctctgagcagttaccgctgaactattgttttccacaactgcaaaacgaagaaatacaagatcttcgaagtgaacgtggaacagaaactgctcgttccacatggggttcagggtgtttcgatggatgggctttgtgcggaaatggcagctgtccagaggcatgcccaggacgtcgacttcaatgcacgggcttcccatgctattactggggcacacattctgaccagagacaatagttaaagaatagactgcaggatccatgctgtccagatctctttctagtggagaaaacttctgatacatggggcagttcttgtcccacagaactggaggtttcaatacataaccacaaccaccatttgcctcaaacattgcagcatttaaatgtaaagggagatcatcagtctggtagttgagtgccacaagctgtatcccatggagccagaacatgagggggttcgggttggaagagtcgatgcgggtggcagcagggtaagttctcagcagctgacaggcggtgtgctgggtcagtttctgagaatacctgcgacacagacgtttggcggcattttcattcagcgacgagatatgataacatttgggagttctaatgatagcactgagggacgtggttgggttgagaggggaagaagattcctcccaggtctgtcgaatgccttcacaggaactttttccagatgttttgttaaatgatgctgtctcccctgggctcattctgcccggattgttgccaaaaatggacttcctgcttttcctttcttttcctctgctagagccagatgcatttagagttgacagtcctggaaattttactgcttgacaatagattacaaggtcagaaagctctggtgcaatctgtctgctttcctttttattctgatcaagataaaattcttctcccagttccatatcataaacctttcctttgttgcaagcagagttatctgctttctttatcctctttgggatttcttcattatattcaaactgaagcttgtcattacatgatttattttcaggtctgtcttccagaatgttgtcatcagaaagggattcatagtcataatcatattcgtcctcctcatcttcctcttcctcattattggcaggtcgggggttggcattcccaccattataagcctgcacttgcatagatgctaactgatgagccttttgctttaagatatccactggcgtctgatgggcttttagcttcttgtttttaagaagaactttctttctgagttggtcaggtgaaggaagcattggatcatctgagaaatcagtctcaaataagaatttagtcaccagcttttctccaaacacagtcttgaaaatttctgccatttttcgttgctgaggcaatgaacagtggttctcaatcgatatgatgattggcaggtcagagttgatgaaggcactgcgatcaatggcttcaaccacttccttgaaggggatcttggttgtcagcgtatgtccatgataaatgatgggcatcccatcgtctccgtcccagcagtccaattctacacttcgacagccttgcaaaaggacctggctgtagagttctaccgaggattctcctttgagctgatggcccgtgaggtaggtattgtgcgaagattcgatgtaatagtatgagaggggtagctgcagttctttaatgttctcctgtgactcatcattttttgaggcaaaattttctttatccatcagaaacctggcaaacccttcaaatgacattagtccctgatgacacatactgatgctaggctcgaacttctggatgatgctgaggatttcatcataagtgcagtgttctccttggcaattcacgaggaaatcgttgagctgaagtatgcccaccccaaaaatgcccagagatgtgctctcaatcccagtgccatttgtcacaatgcttgcagcagcaatggcatcagatatctgcctctggttgtccgatagctgctgtttactcttaatgaacaaccccaaatccgagacatttctggtcaacagatctaggtcaggctgaagatcgctggtgttttcatcaattgtcaggttggtgtagagtggggctgactcggagccagatcggttgcagggcactgcatagacatcaaacagatccttcaggtccttgcggctcctgacactgaatgatttgaacagctcaacaaattcaacaaaactcatgttgctatctgaaaccatgaagctctgaaatcccttcatgccgcctttgatccgcccgtgccagctactactgctccaagcactgatgggagatgacgtcccggcagccaagttgggggacccagctgtggtcaaagagtgggctcttctggaagggagggggtttggagggttagcgatggcattcacctctgattcttcttgttcattaatgtcttgaggatcagaaccactccggcttcgacactctttgtgcatcttggcctttcgggttgccatctcatcgtcagttacctctccactctcacccctcatgaggattttcttctttttcttggtagtgcttatgcccagggtattgtttctctgcatattgggcttctcagcattctttgctgatgttccggggctggggtttcgagcactccaccgtctgccaccaaacaactccacagcgtgagccaaagttgggccttcataccgtccatcctcctgataaaggctgacgtactgtttccgcagccactgctgtctttggtcagggaatttcctcatctttctcacagctctagtgagttccaataatccgctgaagagcattttagctgtgtgctttggtgccacgaagtgcaataatctgttgtctgtggtctgaagcccatagagcaatgtcacaccagtctctgacaggaacatgctacccagtttgttctgaacacacacagtgtgtatatcaatgccagggtggcccatgtatacagccttcactgcaaaaagatccaagaccccttccgtcaggctacttaatccagcattacccagtagtgggaattttccaggctcagctgtgttattaagtacaccaagttttgctttactgctggctggggaggcagttgtgggctttacccaggtcaaggtgctattgtcgggctgaagctggaggaagcagcgggcagagaggtgtgtgtcctggtcgtagtggatgaccgtggccccctgcagcaggaactggtgcacatcggcttggatggacagcacgtaccaagggatgagctccgtcccatggtcgaaggccttctgtgagtcctctgaaccatgagagtcgtattctttggattgctcaaagatgtcattgtctgaatccaacaaatctccaattataaactgccatcggcttttatccttcaaggagcttttcctggagctgtttccttcactggggctgtcctcctcgtctgtctccagacttcgattgcagctccggatgacctgaaagatgctgttgacagtggactccttctccgaattctttaagccattttgtcccactcgttgtaagaaattatcttgtccactgtaatctgctacaaactctaaagtttcttcttgggaattgtaccgcgggcaaagcttcatgagaccggaggcgccgtcaagcacttcacagagctccttcagaaacaccccacagaatggaaccaccttacagccagggatgtgcagggcacgtgtcaccacctttctgtactcacaagaggactcatgctgggccatagcatccttcaggctcctcatggtctcaatatcagactggtccatgaactgccacatttttaaaacttttcttgacctgaggccagccaagaactccatgacagcgttgtagttgcccatgttccagcagcatttggccacatgcaccaaatatgaaaagacttctcgcttctcctccatggagcctgccgtgaggatcagccatgtcacccaggagctcacctcattaaacctcatcaccagatcttcaagggcattgtgctctccattctgagtggtaagaatcgacgctgagatggatgctttgaggcagggcaaggagctctggcattcaggagtgcccaagtcccgtgttaagaagcaaaggtagtcgactggcaagaccctgcggtaaatagtctgctcttgctccatcaggatgctggcgacttcctctgggaactggatgagaggctgcagatcgatcagctccttgctgatcccagctgaacttgaagggagggcattggaattggccacagaggggcctggctggcgttctttcagcatcattcgtccagtggatcctccaaaagtactgagaaggccacttcttgctcccaaagacgtggttgcttctaggagagaaccggtgatgtactgcgatattgaagtcctttggagggtggcgcgatactcacatacagtgtctcggacacattgctttaagcatggaccaacgcttatccttccatgggctgtctcggaggctgggagcttggtgaggaaatggagtagagatccaactgtattttctgtttcttctcttctcactgcattgtagataggataccactgggcttctgacagacgttggctcccatcttgccttatctccactgttgacgggggttccattactctcccacaaggcagtaagggaccatttctcttctgatctatgtaactccatgcagtcagcccaatgtggccagaaggcagagttctcacaattgctcttgttccagtatacacagatttcttaacttctctgtcatttttacagaatctcctgactaacaaagtggatcgctcctttttgcttttaaaagcgtcttcttctacatcatcacaattatcagggaagtcctcaaaatggctcaaaaaggtcttggcagcttgactgtcagtaaagtctttcctacaaaagctatcacctgaatataccatgtcaaccttctcacaagagccttcaaagcaaaagtatttatcattcaaggtgtcacaatgatcacactgcagctgctcattcttattatcacaatttttggccaattccatcagtttacaggtatatgccacatagtttttcttttgcttctcctcacccccaggtagtggtacacaatttccacaatcgtctaaaattaagttttctgatagggtacagaaagtgtctgacattcttctgtcaacttcataatgaaaatgaaatactgcccttctgctgtcagggtgtgctctgcctgtctctatgatcactgactgatttcctaaaggactaatgcccatggaaggtctgtctagttccagttgaattccagggaacacctttctttccagtggagaaggaattccagtttctaaacacaagtcttcctcagcaacagagttgtacatttcataaaattgtctctgaggaaggccatgctgatggtttctcaatatgttgttgcagttaatgttaaggtttttcgcagaatctggcatgattttctcccaacatttttcattactgttctcatcactcactattttctccctcgctattgagagaatctttggcaagttgcttccagaaggttcttctttaagtttgttcagttgtgagatggtatgagaagtctccccacttcgtctgacagtatgtgcttttgaaatattgatgtctgagaccttttcactactttcatctgcagccgactgggcagaaaccacttttctctgagtcacaggtatgagaacagaagctgtcatttcttcagaagtcatcttggactaacacacaggttttgactattgctctatttttcctccctggtgatcatgtcaaggttttaataaaatgactgattattacaacaatctcagatacacaagtcctcccaaagaacaaagggataattcctttcattcaggagcattaagaggcaaataaattttcttagttataacttcctatcatgaatatatattttttctagatcagggttttaaggtggtagatcaattttccttcctctgttacctgaagcaaaattttttgaagacttttactcgggattgcactctgcaacttctgatccatcactgatttgcaatgattttaaaatccagtttgaatgattcctgtttcctcttggctcctggcgagtctcgccggcgtccccaagcgcagcgtccctctgggaccagccgtccgcgcgcctgtcgctagcggcgtcgggtgtccccgctactgtgtgtcagctgcagagccgatgcccaggaacgcgcaggagccaggcaagtgcccgagaggcagagcccgggaggcagagcccgggaggtagagcccgggcgcgccgccgctgcccctcccgccgcgcgagcccgccgcccgccgcgttgcccacgttgcccagcgttaccgtgtggacccgcgccgttcacagtccgctcccgccgagatgtgcgcgctgccc

SEQ ID NO: 15572 - RNA, 10090 nt, Homo sapiens
  source 1..10090: mol_type = other RNA
gctgggattacaggcatgagccactgtgcccagccaactctttacattttgaaacaatgtgttctttctgtaatcccaaagactcaaatacaatgaagtatgtactttcacctcaaaatgtgataaacaactaaattgggatgcaacctaggcagtaggctggattctctcacttgctaaacaacctggtctcaacttcagtctcagatttatgttgtaaaacatacacctgtgttaaaggtcatggaggaggagtggggcagcgcttagcatcagaatcaaatgtgataaacctaaagagacgagtcttttcatcttgttactctgcacagttttcatttggcctctagccacttagaccagcaactcagttttcaacacgtggtagggcaaactgtttggcatgttcacttatagaggcttgataaagtgtttccggaatatttttaaaatggagcagcattgtgcatttgttagaatgaatatttgacttaaaactgtactactgtatagattacatcaaactggaatagcctgaattctgttgacaagaaaatggtagttctagccttaaggctttgacccagtaagaactttcaatgacatgaaagctgtatggtgtttttttttttttttttttttttttttttttttttgagacggagtctcgctctgtcaccaggctggagcgtggtggtgcgatcttggctcactgcagcctccacctcccaggttcaagtgattctcctgcctcagcctcccgagtagctgggattacaggcacgtgccaccacgctcagctaatttttgtacttttagtagagattgggtttcaccatgttggccaggatggcctcattctctgtcctgatccgcccatcttggcctcccaaagtgctggagttacaggcgtgagccactctgcccagcctgtgtggtgtatttttaacacttctgtttttagaatatgcaagaaacacatggggatggttttatttttataattggttaaaaaagtttctcaaagtgaagtttaggagtgagttttagtgttttgtaatttgaagaaaagtgtcttaaaattcaaagataccaatggaaagataaaagtttgggttttagaggaatacatatttcatttttaaaattcataatttgcttcatactaagaatatgaagaatcctttacacttaatggttttgtacagcaaagtttaaaaataatttacattaaatggcaagtatgacttggatcaatagctcttcagttaatgagaaatgaagcaattttacttgaaagtctagcccatttcagatgttcagagcatatattttctttttagaagtttgtcttcaagtactgagaactaatgcttctaatccatggcaatatcaagagagcgatgtataataaatatataagtatagtgtcagtacaaaccttgcaaaataaatttaaacgccaactcaatctacttttgctttaaaaaattgttaggtttcttgttaagacattgcaattcagtagatattaaattatacgtcattctaaattcattttgaaaaccaaaaatgagtaatctaatctatgattaagcaataaccttttttaaagcaaccctattaactgaataggcaataaccttaaaaaaaacccaatattatttctatatgtaaaaaaatcctaaagaggagtgcactgtggtacacaatacaggaactaaattgaattttaatgactcttatgttataggacatatttacacttgaaatgccccaaagcttctaattctaagcttctaattctcggccataaaatgtatggctaaacttcctttcctgttttcagatctttgtgctccttgttcccagttctcttctcttagttgtgttggcaaattaaggtccttgggccaaatctagcctgccacctgtttttgtatggcccctgaattaagaatagtttttaagtttttaaatggttgaaaaaaagtcaaaacaagagtatttgtgacatgtgaaaaatatatgaaattccaatttcagtgtccataaataaagttttattggaatacagccacgttcgttcatgtatgtgttgtctatggctgcttttgcactacaatggcagaattgggtggttgcaacatattttatggcccccagccctaaaatatttactgtttggccctttacagacaagcttgctgacccttgctctaagtcaattcgtgacgatttttccaactgctgacatttataaaatggcagtcccctgggcttcattcatcagtaaattggttggtggcaactagccctgtgccattttgcttctcctcagcatggatctcacatgtgtgaaggcttcagttcagaaatcatcaatttccagtttaagtctgatgaaaataattatattttttccaccatgttcactctttaacttcttgcttaaagatcttcacctgggttaaacatgctgcccttagtcactgtcggtaatccattgtgtcactggaggacaagccacccacaggtttctcctccttggtttggatactttctgaggtcaagagctgagaaggtgatgtaagtcctcggggctgtttagttgacttggtgagcttcttgagttcacttgcgaaagaaatgcctttctttttatcttctcgagatgcctgcacctgctcctttagcttaaggatgaattttcctgcacctttccacttgctttgggcttgaaacacacactcctgatccagaaggacccgctgagaggactttggtgtggtagtcttcttgttggtagtgtctttcaccacctcttccaaaagcacatagtcgcttggattggggttgctcaggatgctgtaggaatatttggctttgcataaggtctgctgaatgacatcctgtgcagtgctgacgcggggtgctttgatgactgttcgaggttgctctggagaaacatcatgcacttggacaaagaaactctcctcctctgagctcaagatcacctctttgtcatcttgaacaatgtttttctcttctaggttttcctgctgggtttttaagacaatcctgcccatgtatccctcttctggaaaccagctgcttaaaatttgcatgatctcctcttctggaccaatggctctctggaatggttgtttcctacattcattcttttctttagatataaaatatttttcttccatcaaaaaatagtctgtggtaacaggtttgatgtcttgttcatttgtcagaatttgctgcagaagctgctttgccttggtgcctccattaatagtgaaaacggtaaagggctctggccctgggaccccatgcaccgtgactctgtgagtctgcaaacattttctttcttctgtattaaacatcgaagaggctgacatggtattgccagaggaattttcttccatccttctgctgttaatgaataaactagaaatctccaagacttcattgtgaaggtttcgcagctgaagatgtcgatatcctcgttttaaagctttcagtggaatgattctctgagcagttaccgctgaactattgttttccacaactgcaaaacgaagaaatacaagatcttcgaagtgaacgtggaacagaaactgctcgttccacatggggttcagggtgtttcgatggatgggctttgtgcggaaatggcagctgtccagaggcatgcccaggacgtcgacttcaatgcacgggcttcccatgctattactggggcacacattctgaccagagacaatagttaaagaatagactgcaggatccatgctgtccagatctctttctagtggagaaaacttctgatacatggggcagttcttgtcccacagaactggaggtttcaatacataaccacaaccaccatttgcctcaaacattgcagcatttaaatgtaaagggagatcatcagtctggtagttgagtgccacaagctgtatcccatggagccagaacatgagggggttcgggttggaagagtcgatgcgggtggcagcagggtaagttctcagcagctgacaggcggtgtgctgggtcagtttctgagaatacctgcgacacagacgtttggcggcattttcattcagcgacgagatatgataacatttgggagttctaatgatagcactgagggacgtggttgggttgagaggggaagaagattcctcccaggtctgtcgaatgccttcacaggaactttttccagatgttttgttaaatgatgctgtctcccctgggctcattctgcccggattgttgccaaaaatggacttcctgcttttcctttcttttcctctgctagagccagatgcatttagagttgacagtcctggaaattttactgcttgacaatagattacaaggtcagaaagctctggtgcaatctgtctgctttcctttttattctgatcaagataaaattcttctcccagttccatatcataaacctttcctttgttgcaagcagagttatctgctttctttatcctctttgggatttcttcattatattcaaactgaagcttgtcattacatgatttattttcaggtctgtcttccagaatgttgtcatcagaaagggattcatagtcataatcatattcgtcctcctcatcttcctcttcctcattattggcaggtcgggggttggcattcccaccattataagcctgcacttgcatagatgctaactgatgagccttttgctttaagatatccactggcgtctgatgggcttttagcttcttgtttttaagaagaactttctttctgagttggtcaggtgaaggaagcattggatcatctgagaaatcagtctcaaataagaatttagtcaccagcttttctccaaacacagtcttgaaaatttctgccatttttcgttgctgaggcaatgaacagtggttctcaatcgatatgatgattggcaggtcagagttgatgaaggcactgcgatcaatggcttcaaccacttccttgaaggggatcttggttgtcagcgtatgtccatgataaatgatgggcatcccatcgtctccgtcccagcagtccaattctacacttcgacagccttgcaaaaggacctggctgtagagttctaccgaggattctcctttgagctgatggcccgtgaggtaggtattgtgcgaagattcgatgtaatagtatgagaggggtagctgcagttctttaatgttctcctgtgactcatcattttttgaggcaaaattttctttatccatcagaaacctggcaaacccttcaaatgacattagtccctgatgacacatactgatgctaggctcgaacttctggatgatgctgaggatttcatcataagtgcagtgttctccttggcaattcacgaggaaatcgttgagctgaagtatgcccaccccaaaaatgcccagagatgtgctctcaatcccagtgccatttgtcacaatgcttgcagcagcaatggcatcagatatctgcctctggttgtccgatagctgctgtttactcttaatgaacaaccccaaatccgagacatttctggtcaacagatctaggtcaggctgaagatcgctggtgttttcatcaattgtcaggttggtgtagagtggggctgactcggagccagatcggttgcagggcactgcatagacatcaaacagatccttcaggtccttgcggctcctgacactgaatgatttgaacagctcaacaaattcaacaaaactcatgttgctatctgaaaccatgaagctctgaaatcccttcatgccgcctttgatccgcccgtgccagctactactgctccaagcactggatgggctcttgtttgaagaagacagcacaggggaggacactggcctgatgggagatgacgtcccggcagccaagttgggggacccagctgtggtcaaagagtgggctcttctggaagggagggggtttggagggttagcgatggcattcacctctgattcttcttgttcattaatgtcttgaggatcagaaccactccggcttcgacactctttgtgcatcttggcctttcgggttgccatctcatcgtcagttacctctccactctcacccctcatgaggattttcttctttttcttggtagtgcttatgcccagggtattgtttctctgcatattgggcttctcagcattctttgctgatgttccggggctggggtttcgagcactccaccgtctgccaccaaacaactccacagcgtgagccaaagttgggccttcataccgtccatcctcctgataaaggctgacgtactgtttccgcagccactgctgtctttggtcagggaatttcctcatctttctcacagctctagtgagttccaataatccgctgaagagcattttagctgtgtgctttggtgccacgaagtgcaataatctgttgtctgtggtctgaagcccatagagcaatgtcacaccagtctctgacaggaacatgctacccagtttgttctgaacacacacagtgtgtatatcaatgccagggtggcccatgtatacagccttcactgcaaaaagatccaagaccccttccgtcaggctacttaatccagcattacccagtagtgggaattttccaggctcagctgtgttattaagtacaccaagttttgctttactgctggctggggaggcagttgtgggctttacccaggtcaaggtgctattgtcgggctgaagctggaggaagcagcgggcagagaggtgtgtgtcctggtcgtagtggatgaccgtggccccctgcagcaggaactggtgcacatcggcttggatggacagcacgtaccaagggatgagctccgtcccatggtcgaaggccttctgtgagtcctctgaaccatgagagtcgtattctttggattgctcaaagatgtcattgtctgaatccaacaaatctccaattataaactgccatcggcttttatccttcaaggagcttttcctggagctgtttccttcactggggctgtcctcctcgtctgtctccagacttcgattgcagctccggatgacctgaaagatgctgttgacagtggactccttctccgaattctttaagccattttgtcccactcgttgtaagaaattatcttgtccactgtaatctgctacaaactctaaagtttcttcttgggaattgtaccgcgggcaaagcttcatgagaccggaggcgccgtcaagcacttcacagagctccttcagaaacaccccacagaatggaaccaccttacagccagggatgtgcagggcacgtgtcaccacctttctgtactcacaagaggactcatgctgggccatagcatccttcaggctcctcatggtctcaatatcagactggtccatgaactgccacatttttaaaacttttcttgacctgaggccagccaagaactccatgacagcgttgtagttgcccatgttccagcagcatttggccacatgcaccaaatatgaaaagacttctcgcttctcctccatggagcctgccgtgaggatcagccatgtcacccaggagctcacctcattaaacctcatcaccagatcttcaagggcattgtgctctccattctgagtggtaagaatcgacgctgagatggatgctttgaggcagggcaaggagctctggcattcaggagtgcccaagtcccgtgttaagaagcaaaggtagtcgactggcaagaccctgcggtaaatagtctgctcttgctccatcaggatgctggcgacttcctctgggaactggatgagaggctgcagatcgatcagctccttgctgatcccagctgaacttgaagggagggcattggaattggccacagaggggcctggctggcgttctttcagcatcattcgtccagtggatcctccaaaagtactgagaaggccacttcttgctcccaaagacgtggttgcttctaggagagaaccggtgatgtactgcgatattgaagtcctttggagggtggcgcgatactcacatacagtgtctcggacacattgctttaagcatggaccaacgcttatccttccatgggctgtctcggaggctgggagcttggtgaggaaatggagtagagatccaactgtattttctgtttcttctcttctcactgcattgtagataggataccactgggcttctgacagacgttggctcccatcttgccttatctccactgttgacgggggttccattactctcccacaaggcagtaagggaccatttctcttctgatctatgtaactccatgcagtcagcccaatgtggccagaaggcagagttctcacaattgctcttgttccagtatacacagatttcttaacttctctgtcatttttacagaatctcctgactaacaaagtggatcgctcctttttgcttttaaaagcgtcttcttctacatcatcacaattatcagggaagtcctcaaaatggctcaaaaaggtcttggcagcttgactgtcagtaaagtctttcctacaaaagctatcacctgaatataccatgtcaaccttctcacaagagccttcaaagcaaaagtatttatcattcaaggtgtcacaatgatcacactgcagctgctcattcttattatcacaatttttggccaattccatcagtttacaggtatatgccacatagtttttcttttgcttctcctcacccccaggtagtggtacacaatttccacaatcgtctaaaattaagttttctgatagggtacagaaagtgtctgacattcttctgtcaacttcataatgaaaatgaaatactgcccttctgctgtcagggtgtgctctgcctgtctctatgatcactgactgatttcctaaaggactaatgcccatggaaggtctgtctagttccagttgaattccagggaacacctttctttccagtggagaaggaattccagtttctaaacacaagtcttcctcagcaacagagttgtacatttcataaaattgtctctgaggaaggccatgctgatggtttctcaatatgttgttgcagttaatgttaaggtttttcgcagaatctggcatgattttctcccaacatttttcattactgttctcatcactcactattttctccctcgctattgagagaatctttggcaagttgcttccagaaggttcttctttaagtttgttcagttgtgagatggtatgagaagtctccccacttcgtctgacagtatgtgcttttgaaatattgatgtctgagaccttttcactactttcatctgcagccgactgggcagaaaccacttttctctgagtcacaggtatgagaacagaagctgtcatttcttcagaagtcatcttggactaacacacaggttttgactattgctctatttttcctccctggtgatcatgtcaaggttttaataaaatgactgattattacaacaatctcagatacacaagtcctcccaaagaacaaagggataattcctttcattcaggagcattaagaggcaaataaattttcttagttataacttcctatcatgaatatatattttttctagatcagggttttaaggtggtagatcaattttccttcctctgttacctgaagcaaaattttttgaagacttttactcgggattgcactctgcaacttctgatccatcactgatttgcaatgattttaaaatccagtttgaatgattcctgtttcctcttggctcctggcgagtctcgccggcgtccccaagcgcagcgtccctctgggaccagccgtccgcgcgcctgtcgctagcggcgtcgggtgtccccgctactgtgtgtcagctgcagagccgatgcccaggaacgcgcaggagccaggcaagtgcccgagaggcagagcccgggaggcagagcccgggaggtagagcccgggcgcgccgccgctgcccctcccgccgcgcgagcccgccgcccgccgcgttgcccacgttgcccagcgttaccgtgtggacccgcgccgttcacagtccgctcccgccgagatgtgcgcgctgccc

SEQ ID NO: 15573 - RNA, 1429 nt, Homo sapiens
  source 1..1429: mol_type = other RNA
gctgggattacaggcatgagccactgtgcccagccaagcctatgcttttaaatgtcgcattatcctgcatggttagaagaatcatgaccaagtttgtggtcagtggggaaaactgtacttctgtgctctaagcgctacgtcaaagagctctggaatgtccaggctccagacttccaggcctcagctggccgtggtacccctctgcacagatgtctccactatgagccttcaactggcaaggacttaccaaaagcaactatgtgccaggctagggtgtggagcagacaggatgcagtctctggcctgtaggactcagagtccagagagggagacaagagagacccagaggacagacacttagcagaggctgggaatgctccagtgagggaagagtggccacgggcctgagcagtcctccagtgctttgtgaccaggataaataagtcgaggtggagtggtgcagaggtcccaggctttttaagccctaaggttcaatcctggctccagcccttatgagctgtgtgatctcaggcatgtggcatgagcctcattttcctcatctacggtttcagagggcgcacaccgggccttgtggttgtgggtgccgtttcatgctggggttcgcgtccctcctctgtttggcataaagagagtggaacagatcaggccctcagatctgtgtgcacctgcggtcgctctctgggctgctgtgaggatgagatgagataacacacaggaaggtgttctcgctacatgagtgttcccagtcattcttagggccaagaggtatttactggatatctgctctctgccaggacctggctctgcccaggggacccagtcatgagcaagacggaggagtctcagctggagggaacagggctgcagtttgccatcgaagtcactcagcaaattagtcagaggaatctctccggcctgagagggaaggggcccttcttggcccacccctccttcctctgccggctgatgtgttgttggtcaaaagtgatccagtagacgcttcacctctgtagagaggctgccagccctggaataggcaggcccgagtggtggagagccccggtcctggagacagaccatcctgagtttcaacctttgctctgccttttactagctgtgtgacctcaggcaaggaacttgaccttcttgggtccactttccctaataatagtcattccaagctcatgtggctgtggtgaagaccaaacaaggtaattgatgtgaagccccttgcataatactaggcatgggtgagctgggaagttaatttgtgtatatttaacaaacacaggaccacaaactcttccaactacgttaaaaacagtaaccatttaatccttacaagattccagtgagacaggcagtgttgtcatcctcttttttttttttaaatggagtctcatcctgt

SEQ ID NO: 15574 - RNA, 2890 nt, Homo sapiens
  source 1..2890: mol_type = other RNA
gctgggattacaggcatgagccactgtgcccagccacaaataatttatctaagaagtgtttccaaactcattacatttgcaggaatcttcttcaatatacattccctgatgttgcacaaagtttggcaaccgctttagggtttccttctaatacaaaacgcgggcaataagatctgtaatacaagcaaaggtactacaaacctctttatatttgtaatgcttgtcttcagaatcaatactcttcttcaccttaaaggcttatattttctgaaagatttttgtcacagtaattgctcttttatgaaccttcttctgttgagtaagatgtgatggacattaatggcttttccatattctttatatttgtacaatttttctcaaggataatagctttcctgtgaaatacggtgtaagcactgattaaaagttttgccacattcttcatacttgtaggtattttggaagtatgaattacctacaataaagtgtggcaaccatataaaggctttgtcacatttcatacatttctatggtgtagtataattttttttatgcatagaaaagttggaggtgttgggaaaagcactgtcacatctttcaggtttgtaaagttcctcttcaccatgaattatcgccatgtctcttaagaattaagagcttatggctgggaattgaggctcatgcctgtcatcccagcactttaggaagccgaggcgagtggatcacctgaggtcaggagtttgagaccagcctggcaaatatggcaaaagcccatctctactaaaaatacaaaaattagctgggaatggtggtggcacctgtaatcccagctacttgggaggctgaggcaggagaatggcttgaacccaggaggcagaggtcacagtaagccaagatcatgccattgcactacagcccgggtcacaagagtgaaactgcatctcaaaaaataaataaacaaataaaaataaaagaattgagaacttgttacaggcttgccacattcttcacacttgtagggtttctgtccagtatgaattatgtgtaataagggttgagaacttccttaaaaagctttgtcagccaggcacagtggctcatgcctgtaaccccaacactttgggaggccaaagcaggcagaccacctgaggttaggagattgagaccagcctgaccaacatggagaaaccccatctctactaaaaatacaaaattagccaggtgtggtggtgcagccctgtaatcctagctactaaggagagttacttgaacccagaaggtggaggttgtggtgagccaaaattatgccattgcactccagcctgggaaacaacagcagaattacctctcaaaaaaataataataataaaataatcctttgtcacgttcttggtttctgtccaatatgaattctcttatgtttattaaggtctgaggaccagttaaaagctttgccacattctttacatttgtaaggtttctctccagtatgagttgtcttatgttcagttagatttgaggatgtagtatacgctttgccacattcttcacatttgtagggtttctctccagtatgagttctcctatgtttatggaggcctgcagaccatgtaaaggctttgccacattcttcacatttgtatggtttctctccagtatgaattatcttatgcatagtaaggtgtgaggagcgggtgaaggctttgccacattcttcacatttgtagggtttctctcccgtatgaatcttctcatgtttactaaggatcgaggatgaaataaaggctttgccacatttatcacacgtgtacggtttctctccagtatgaattttcttatgtgaagaaagagttgcaggatggttaaaagctttgtcacattctttacatttgtagggttgctctccagtatggattatcttatgtgtagtaagggtataggggtacataaaggctttgccacattcttcacaaatgtagggtttctctccactatgaattttcttatgtgtagtaaagctagagaagtacttaaagactttgccacattcttcacatttgtagggtttctctctagtatgagttatcttatgtgtagtaaggtgtgaggaccggttgaaggctttgccacattcttcacatttgtatggtttctctccagtatcaatttttttatgtgtagtatgggttgaggactggttaaaagctttgtcaccttctatatatttcaaaggttttttttcagtatgtcttcttttatgtctctttgaatttgaaaattgatgaaagactttcacatatttaccacattgaaatattttgctctgggtagttgtcaaacattggttaagtccattataacctcttttgtgtaacttacactcatccacactttcacagccttttttaaagtgtaaattgccatgtccacatttttcaaattttctcagtatcactttttggtaagaatcttttatgctctgctctggccaaaggtcttgggcaaaatgagaacacacaactgggggtttggcaatcatctcatgtctcttcatagtcagaggttttattccttgctccagacaggtgatcaggtctggcttagagacaataataccaaggaagaccaggtgtctgtagttctctaacatcacatccctatataaattctgctgtgcagtgtccaggcaatgccactcctccagagagaattctacagccacatctctaaattgcaatgattccatttctaggcttctaaggggtcccggcatcttggctgtggatctcccaatacctacaggacacagggccacagagggtgggcctctaggagcagaggacacagagtagcgaagaggcgacctagagctccagatgcagcgagagac

SEQ ID NO: 15575 - RNA, 5023 nt, Homo sapiens
  source 1..5023: mol_type = other RNA
gctgggattacaggcatgagccactgtgcccagccagaaatgttaaactcactttatggtttcagaacaaggatcaaataaaataaaaatataaaaaataaaatatggttggccaagtgtggtggctcagccctctaatcccagccctttggaaggccaaggcagaaggctcgcttgagctcaggagttcaagactagccttggcaacatagcaagacctcatttctgctaaaaataaaaaacattagccagacatggtggtccacacttgcagtcccagttattcaagaggctgaggtgggaggatcacttgagcttgggagatcgaggctgcagtgagctatcatcgtgccactgcactccagtctggcgacagagcaagaccttctcaaaaataaaatatggtcgaaacgggacagacaaggcggctacctgtaaccctggccgctttaggagctggggcaggaaagttgcttgaggccaggaatccgagaccagcctgagcaacagcaggacccgtctatgaaaaaacaggagcaagtagtggcacatcccaattgtgtcagctaactgggaggctgaggcaggaggatcgcttgagcccaggagttcaaggctgtactccagcctgggcgacaaagcaagaaccctgttctctagggaaaaaaaaaaaaaagtcaaaacatttcataaaactttcacacaatggaggtttagttaagctgttactcttctgttcaattttgttgcacctatcagaaggcataatttcataaaatcaggattccttggcgttttaaccactctcaaaatatttgatcctactggaagttactatgcaatgctatcttgtccctgaatcaacataattcaactatcagcttcatatatatatatatatatatatattttttttttttgagacagagtttcgctgttgttgcccaggctggagtgcaatggcgcaatcttggctcaccacaacctccgcctcccgggttcaagcgattctcctgcctcagcctcctgagtagctgggattacaggcacgcaccaccaccgcagctaattttgtatttttagtagagacagggtttctccatgttggtcaggctggtcttgaactcccgacctcaggtgatccacccgcctcggcctcccagaatgctgggtttacaggcatgacccactgtgcctggcagtttcgtgtattcttactccactgggttctgctttatcgtattgacagtagacatttcattaaatgaaatgtaaaaagaacaccaatacatacatattaaaattttcttactagaatcttttagtataatttaaaaacctgaaatgagaattcgcatcactttaagtgggcctcttgggttttgaggatgaagtggctttctctcagaaatagctttgaaccgtaactctagtaactacagtggcaggctccatagcttgaacacagcgtattttgtatcaatgcccacaaataaaacctattataactcttaggaaataaaacttgaatcctgattggcagaactgcctcagtaagggctggctgaactgcatacccaaaatgttttagatctacggtccactttcacgttggctggactaatgcgtttctactgctcctcttacacgttgactgactttcctctcaggaagaggtagagactatgttccttttttcctcaatctgggacttggtttctgagacatcactgttgtaaccaagagcatggtaaaagtgatgttatgtgacattgaaggataagtcctaaaaagccaactctgccaagctctcctggagccccaaaataccacctaagtccagctgccctgaagccaccatgctagagattttcgggaaagactataccactaatagtgaaaagcacaaagagcatcctttcagctcagaagtgaaaagcttcatgagactcagaaccagaagagtctgatactcccgagttcttcacccacagaaaagcttatcatacaccattgatctttggatgctttgctaacatagcaagaaataatatacagttgatactgctaagcaccacagccaccacttggttgggttcagaagacatcctactttacctttttaaagtttggtccaaatttgtacctacaacttttccttttttcctgcagcacaggtaaaatgttggaacctttaacaagttcaggcaatgatgatataaagaagttaacatgcaactagctgcactggcttctaaattgagttcactgaccttaccatgagtttgtagtaacatttctctccaatctctgaaaaagtttttctctccaggccatctgtacgctttacgtagggactgttaaccaacccacgtattacacataaggactctaggtaaaatctagtgtttgaaaaacagcatgttatatattacactaggtttttcgttttttttccagtggtgggctgtcattacaaaagattgaacttttatacacttcctaatcaaacttaaggggaatctaaacacaaaaactaattcactttctaggagctctttaaaaatgggcttaaacctacaatccaatctcgtatctaagtatgatggaatgctttttccccagtggcattcatatagttcagctgtcaagcagtacctttcttaaaataccagactgaaaatagttcaattttctgtaaaaagtcagagccgggcacggtggctcatgcctataatcccagcagtttgggaggctgaggcgggcggatcacctgaggttggaagttcgagaccagcctgaccaacacagggaaaccccgtctctactaaaaatacaaaattagctgggcgtggtggcacatgcctgaaatcccagctacttgggaggctgaggcagaacaatcgcttgaacctgggaggcagaggttgccgtgaggcgagatcgcgacactacactcgtctgggcaacaagagtgaaactccgtctcaaaaaaaaaaaaagtcagatctgtgtaaagagaattagtgtacctgaaaattgttttcagctgtcaatcactttggtcctttactgtcattctaagaatcagcctaatttggtttaccttgtcttacaaataaggattagcaaactcaccaacataaaaaaggtgtagtacatgctgcaaaaatgtaagtatacactgacatttacttgccaaaataaccacaaatgactacacatatttaactataattaaatcaagtttttagaaatttaaagtctgcttccctagaaatacaggaactttgtgtgataaaacttgagacatatgacaatttctgaatagcaactggaatattcaaccaacaatggtcatggtcagttttgtattttttccttaacttatatacttcattctttccaactattttaaagctaaatcttttttaaaaaagttttaaaaataagtcacaggcaaatcatgaagagttgggtttatttcaacagtaaatctgaaactcttgccttaagcaagagtactacagtaattatatcaggaatagacaatttcctacactgtcaaatatataaaagttccttttgcactttcttcaacactgatcaacaagcagattcagtccacatttgctttgatctaactactgagttaacccaagcttcttcttcagagactctggcatctcgggtggaggagggcgaggaagtctgaagtagaccttcacggagtcatagataaaccactgtagtgcagtcagggtaccaatcatgatgatacgggcaaacagtcccttccatacacctttaaatccaagtctcttgaggaccagagaagcactgctacctttttctttattcaacacagataccacagaatcagcagggtgagaaacaattgcacaaaagactccagctatgtaacctgctacaaatgttacaaccagctgctctggctttgaacattcactgcggggcttaggaaccacaaacttgtacagtgcttcaacagtacgttcaaagcaggcgaacttcatcatggtgtatggtatctgtctcatccagagaggagcaacccccttgtagaatgcttttaggccttcttccttatacattttgggagctgcatccctcaaagtgttggcataacctggctgggtttgaattcgaaccttagcagcttccataggagccagggcaatgtcagcaaagaattcagcactggcagaggcagccaaatatagtgatgtgcgccagagataagtattctcctctccaagcatattgctatacaagactttaaagacttcataaaagccaaacttgcagagtccctgcatggagtagccaaggaaagtcggagcccatcctttagccaaaccacgaacaccatcctctttaagtgtaactgagaatccgttaaatatgcccttgtacttttgggggtccacctgcatacggcatttcactaaatccaggggaaccacagcagtgtgtgtcagaccacaacttaagaccccaccaaagccacacagtgcataatacttcgcggagccaaattcacaactgtactcttccacggcggcggctgccaggttgcgagggcggcggggctggcccgtgggccctggggagctgctgcggaggtccccgagaccatcgtgcaccagctgcagatgtggcgtgttgaaggggttcgcccgcgccaggtgcgccacggacgagaacatctttctaggggaggagggagcgacggttagaggacaggcaaggcgccggttaacgttaccggcgccctggaaccccaaccggggccttttccttcccgtctccacgcccttgaagaggtcacggcggccttcgaaagaggctgctcccggctgggcccaccgccaaagcagcggccccacaggagctctgggctccgctccccacacccgccacaggagaaggcccggccacactcactccctaagatggcgatcacacaaccactcccttggaaaggttgcggctcacagag

SEQ ID NO: 15576 - RNA, 4789 nt, Homo sapiens
  source 1..4789: mol_type = other RNA
gctgggattacaggcatgagccactgtgcccagccagaaatgttaaactcactttatggtttcagaacaaggatcaaataaaataaaaatataaaaaataaaatatggttggccaagtgtggtggctcagccctctaatcccagccctttggaaggccaaggcagaaggctcgcttgagctcaggagttcaagactagccttggcaacatagcaagacctcatttctgctaaaaataaaaaacattagccagacatggtggtccacacttgcagtcccagttattcaagaggctgaggtgggaggatcacttgagcttgggagatcgaggctgcagtgagctatcatcgtgccactgcactccagtctggcgacagagcaagaccttctcaaaaataaaatatggtcgaaacgggacagacaaggcggctacctgtaaccctggccgctttaggagctggggcaggaaagttgcttgaggccaggaatccgagaccagcctgagcaacagcaggacccgtctatgaaaaaacaggagcaagtagtggcacatcccaattgtgtcagctaactgggaggctgaggcaggaggatcgcttgagcccaggagttcaaggctgtactccagcctgggcgacaaagcaagaaccctgttctctagggaaaaaaaaaaaaaagtcaaaacatttcataaaactttcacacaatggaggtttagttaagctgttactcttctgttcaattttgttgcacctatcagaaggcataatttcataaaatcaggattccttggcgttttaaccactctcaaaatatttgatcctactggaagttactatgcaatgctatcttgtccctgaatcaacataattcaactatcagcttcatatatatatatatatatatatattttttttttttgagacagagtttcgctgttgttgcccaggctggagtgcaatggcgcaatcttggctcaccacaacctccgcctcccgggttcaagcgattctcctgcctcagcctcctgagtagctgggattacaggcacgcaccaccaccgcagctaattttgtatttttagtagagacagggtttctccatgttggtcaggctggtcttgaactcccgacctcaggtgatccacccgcctcggcctcccagaatgctgggtttacaggcatgacccactgtgcctggcagtttcgtgtattcttactccactgggttctgctttatcgtattgacagtagacatttcattaaatgaaatgtaaaaagaacaccaatacatacatattaaaattttcttactagaatcttttagtataatttaaaaacctgaaatgagaattcgcatcactttaagtgggcctcttgggttttgaggatgaagtggctttctctcagaaatagctttgaaccgtaactctagtaactacagtggcaggctccatagcttgaacacagcgtattttgtatcaatgcccacaaataaaacctattataactcttaggaaataaaacttgaatcctgattggcagaactgcctcagtaagggctggctgaactgcatacccaaaatgttttagatctacggtccactttcacgttggctggactaatgcgtttctactgctcctcttacacgttgactgactttcctctcaggaagaggtagagactatgttccttttttcctcaatctgggacttggtttctgagacatcactgttgtaaccaagagcatggtaaaagtgatgttatgtgacattgaaggataagtcctaaaaagccaactctgccaagctctcctggagccccaaaataccacctaagtccagctgccctgaagccaccatgctagagattttcgggaaagactataccactaatagtgaaaagcacaaagagcatcctttcagctcagaagtgaaaagcttcatgagactcagaaccagaagagtctgatactcccgagttcttcacccacagaaaagcttatcatacaccattgatctttggatgctttgctaacatagcaagaaataatatacagttgatactgctaagcaccacagccaccacttggttgggttcagaagacatcctactttacctttttaaagtttggtccaaatttgtacctacaacttttccttttttcctgcagcacaggtaaaatgttggaacctttaacaagttcaggcaatgatgatataaagaagttaacatgcaactagctgcactggcttctaaattgagttcactgaccttaccatgagtttgtagtaacatttctctccaatctctgaaaaagtttttctctccaggccatctgtacgctttacgtagggactgttaaccaacccacgtattacacataaggactctaggtaaaatctagtgtttgaaaaacagcatgttatatattacactaggtttttcgttttttttccagtggtgggctgtcattacaaaagattgaacttttatacacttcctaatcaaacttaaggggaatctaaacacaaaaactaattcactttctaggagctctttaaaaatgggcttaaacctacaatccaatctcgtatctaagtatgatggaatgctttttccccagtggcattcatatagttcagctgtcaagcagtacctttcttaaaataccagactgaaaatagttcaattttctgtaaaaagtcagagccgggcacggtggctcatgcctataatcccagcagtttgggaggctgaggcgggcggatcacctgaggttggaagttcgagaccagcctgaccaacacagggaaaccccgtctctactaaaaatacaaaattagctgggcgtggtggcacatgcctgaaatcccagctacttgggaggctgaggcagaacaatcgcttgaacctgggaggcagaggttgccgtgaggcgagatcgcgacactacactcgtctgggcaacaagagtgaaactccgtctcaaaaaaaaaaaaagtcagatctgtgtaaagagaattagtgtacctgaaaattgttttcagctgtcaatcactttggtcctttactgtcattctaagaatcagcctaatttggtttaccttgtcttacaaataaggattagcaaactcaccaacataaaaaaggtgtagtacatgctgcaaaaatgtaagtatacactgacatttacttgccaaaataaccacaaatgactacacatatttaactataattaaatcaagtttttagaaatttaaagtctgcttccctagaaatacaggaactttgtgtgataaaacttgagacatatgacaatttctgaatagcaactggaatattcaaccaacaatggtcatggtcagttttgtattttttccttaacttatatacttcattctttccaactattttaaagctaaatcttttttaaaaaagttttaaaaataagtcacaggcaaatcatgaagagttgggtttatttcaacagtaaatctgaaactcttgccttaagcaagagtactacagtaattatatcaggaatagacaatttcctacactgtcaaatatataaaagttccttttgcactttcttcaacactgatcaacaagcagattcagtccacatttgctttgatctaactactgagttaacccaagcttcttcttcagagactctggcatctcgggtggaggagggcgaggaagtctgaagtagaccttcacggagtcatagataaaccactgtagtgcagtcagggtaccaatcatgatgatacgggcaaacagtcccttccatacacctttaaatccaagtctcttgaggaccagagaagcactgctacctttttctttattcaacacagataccacagaatcagcagggtgagaaacaattgcacaaaagactccagctatgtaacctgctacaaatgttacaaccagctgctctggctttgaacattcactgcggggcttaggaaccacaaacttgtacagtgcttcaacagtacgttcaaagcaggcgaacttcatcatggtgtatggtatctgtctcatccagagaggagcaacccccttgtagaatgcttttaggccttcttccttatacattttgggagctgcatccctcaaagtgttggcataacctggctgggtttgaattcgaaccttagcagcttccataggagccagggcaatgtcagcaaagaattcagcactggcagaggcagccaaatatagtgatgtgcgccagagataagtattctcctctccaagcatattgctatacaagactttaaagacttcataaaagccaaacttgcagagtccctgcatggagtagccaaggaaagtcggagcccatcctttagccaaaccacgaacaccatcctctttaagtgtaactgagaatccgttaaatatgcccttgtacttttgggggtccacctgcatacggcatttcactaaatccaggggaaccacagcagtgtgtgtcagaccacaacttaagaccccaccaaagccacacagtgcataatacttcgcggagccaaattcacaactgtactcttccacggcggcggctgccaggttgcgagggcggcggggctggcccgtgggccctggggagctgctgcggaggtccccgagaccatcgtgcaccagctgcagatgtggcgtgttgaaggggttcgcccgcgccaggtgcgccacggacgagaacatcttttccctaagatggcgatcacacaaccactcccttggaaaggttgcggctcacagag

SEQ ID NO: 15577 - RNA, 4792 nt, Homo sapiens
  source 1..4792: mol_type = other RNA
gctgggattacaggcatgagccactgtgcccagccagaaatgttaaactcactttatggtttcagaacaaggatcaaataaaataaaaatataaaaaataaaatatggttggccaagtgtggtggctcagccctctaatcccagccctttggaaggccaaggcagaaggctcgcttgagctcaggagttcaagactagccttggcaacatagcaagacctcatttctgctaaaaataaaaaacattagccagacatggtggtccacacttgcagtcccagttattcaagaggctgaggtgggaggatcacttgagcttgggagatcgaggctgcagtgagctatcatcgtgccactgcactccagtctggcgacagagcaagaccttctcaaaaataaaatatggtcgaaacgggacagacaaggcggctacctgtaaccctggccgctttaggagctggggcaggaaagttgcttgaggccaggaatccgagaccagcctgagcaacagcaggacccgtctatgaaaaaacaggagcaagtagtggcacatcccaattgtgtcagctaactgggaggctgaggcaggaggatcgcttgagcccaggagttcaaggctgtactccagcctgggcgacaaagcaagaaccctgttctctagggaaaaaaaaaaaaaagtcaaaacatttcataaaactttcacacaatggaggtttagttaagctgttactcttctgttcaattttgttgcacctatcagaaggcataatttcataaaatcaggattccttggcgttttaaccactctcaaaatatttgatcctactggaagttactatgcaatgctatcttgtccctgaatcaacataattcaactatcagcttcatatatatatatatatatatatattttttttttttgagacagagtttcgctgttgttgcccaggctggagtgcaatggcgcaatcttggctcaccacaacctccgcctcccgggttcaagcgattctcctgcctcagcctcctgagtagctgggattacaggcacgcaccaccaccgcagctaattttgtatttttagtagagacagggtttctccatgttggtcaggctggtcttgaactcccgacctcaggtgatccacccgcctcggcctcccagaatgctgggtttacaggcatgacccactgtgcctggcagtttcgtgtattcttactccactgggttctgctttatcgtattgacagtagacatttcattaaatgaaatgtaaaaagaacaccaatacatacatattaaaattttcttactagaatcttttagtataatttaaaaacctgaaatgagaattcgcatcactttaagtgggcctcttgggttttgaggatgaagtggctttctctcagaaatagctttgaaccgtaactctagtaactacagtggcaggctccatagcttgaacacagcgtattttgtatcaatgcccacaaataaaacctattataactcttaggaaataaaacttgaatcctgattggcagaactgcctcagtaagggctggctgaactgcatacccaaaatgttttagatctacggtccactttcacgttggctggactaatgcgtttctactgctcctcttacacgttgactgactttcctctcaggaagaggtagagactatgttccttttttcctcaatctgggacttggtttctgagacatcactgttgtaaccaagagcatggtaaaagtgatgttatgtgacattgaaggataagtcctaaaaagccaactctgccaagctctcctggagccccaaaataccacctaagtccagctgccctgaagccaccatgctagagattttcgggaaagactataccactaatagtgaaaagcacaaagagcatcctttcagctcagaagtgaaaagcttcatgagactcagaaccagaagagtctgatactcccgagttcttcacccacagaaaagcttatcatacaccattgatctttggatgctttgctaacatagcaagaaataatatacagttgatactgctaagcaccacagccaccacttggttgggttcagaagacatcctactttacctttttaaagtttggtccaaatttgtacctacaacttttccttttttcctgcagcacaggtaaaatgttggaacctttaacaagttcaggcaatgatgatataaagaagttaacatgcaactagctgcactggcttctaaattgagttcactgaccttaccatgagtttgtagtaacatttctctccaatctctgaaaaagtttttctctccaggccatctgtacgctttacgtagggactgttaaccaacccacgtattacacataaggactctaggtaaaatctagtgtttgaaaaacagcatgttatatattacactaggtttttcgttttttttccagtggtgggctgtcattacaaaagattgaacttttatacacttcctaatcaaacttaaggggaatctaaacacaaaaactaattcactttctaggagctctttaaaaatgggcttaaacctacaatccaatctcgtatctaagtatgatggaatgctttttccccagtggcattcatatagttcagctgtcaagcagtacctttcttaaaataccagactgaaaatagttcaattttctgtaaaaagtcagagccgggcacggtggctcatgcctataatcccagcagtttgggaggctgaggcgggcggatcacctgaggttggaagttcgagaccagcctgaccaacacagggaaaccccgtctctactaaaaatacaaaattagctgggcgtggtggcacatgcctgaaatcccagctacttgggaggctgaggcagaacaatcgcttgaacctgggaggcagaggttgccgtgaggcgagatcgcgacactacactcgtctgggcaacaagagtgaaactccgtctcaaaaaaaaaaaaagtcagatctgtgtaaagagaattagtgtacctgaaaattgttttcagctgtcaatcactttggtcctttactgtcattctaagaatcagcctaatttggtttaccttgtcttacaaataaggattagcaaactcaccaacataaaaaaggtgtagtacatgctgcaaaaatgtaagtatacactgacatttacttgccaaaataaccacaaatgactacacatatttaactataattaaatcaagtttttagaaatttaaagtctgcttccctagaaatacaggaactttgtgtgataaaacttgagacatatgacaatttctgaatagcaactggaatattcaaccaacaatggtcatggtcagttttgtattttttccttaacttatatacttcattctttccaactattttaaagctaaatcttttttaaaaaagttttaaaaataagtcacaggcaaatcatgaagagttgggtttatttcaacagtaaatctgaaactcttgccttaagcaagagtactacagtaattatatcaggaatagacaatttcctacactgtcaaatatataaaagttccttttgcactttcttcaacactgatcaacaagcagattcagtccacatttgctttgatctaactactgagttaacccaagcttcttcttcagagactctggcatctcgggtggaggagggcgaggaagtctgaagtagaccttcacggagtcatagataaaccactgtagtgcagtcagggtaccaatcatgatgatacgggcaaacagtcccttccatacacctttaaatccaagtctcttgaggaccagagaagcactgctacctttttctttattcaacacagataccacagaatcagcagggtgagaaacaattgcacaaaagactccagctatgtaacctgctacaaatgttacaaccagctgctctggctttgaacattcactgcggggcttaggaaccacaaacttgtacagtgcttcaacagtacgttcaaagcaggcgaacttcatcatggtgtatggtatctgtctcatccagagaggagcaacccccttgtagaatgcttttaggccttcttccttatacattttgggagctgcatccctcaaagtgttggcataacctggctgggtttgaattcgaaccttagcagcttccataggagccagggcaatgtcagcaaagaattcagcactggcagaggcagccaaatatagtgatgtgcgccagagataagtattctcctctccaagcatattgctatacaagactttaaagacttcataaaagccaaacttgcagagtccctgcatggagtagccaaggaaagtcggagcccatcctttagccaaaccacgaacaccatcctctttaagtgtaactgagaatccgttaaatatgcccttgtacttttgggggtccacctgcattctgcatttaaccagatctagaggaaccaatgctgtatgtgttgtgccacagctaataattcctccaagtccacaaaggataaagaatctgccagatccatagtcacagctatactgctcttccacggcggcggctgccaggttgcgagggcggcggggctggcccgtgggccctggggagctgctgcggaggtccccgagaccatcgtgcaccagctgcagatgtggcgtgttgaaggggttcgcccgcgccaggtgcgccacggacgagaacatcttttccctaagatggcgatcacacaaccactcccttggaaaggttgcggctcacagag

SEQ ID NO: 15578 - RNA, 2349 nt, Homo sapiens
  source 1..2349: mol_type = other RNA
gctgggattacaggcatgagccactgtgcccagccagagcctagcttgtaatcactccgctctactacctcccaccttcctttctttgtgtaataagattgcagtacacagtgctgtacaataaacaaaatatttttatacacatagtcacacttcatcctcacagggatcctgaggcaggagaacagttacttttgtatttctccattttgcagtttataaaactgaggctcagaaaaattgaacttctttgcccaaggtcattcaggtactaagtggtagctgggactcaaagcagttcttccaactcaaatccccatttctttctgtattcgtctgcttgggctgccatcacaaagcagcataaaccgggaggcttaagcaacaaacatatctcatctcacagttctggacgctgaagtccaaaatcaaggcatcagcaggattagaactttctgaggggttgagagagactctattccatgtcccgctcctggcttctgggggctgctggcaatccttgcgcattcctcggtctgcaggtgcatcagtccagtgtctgtctccattgtcacatggcattctctccttgtgtgtctctctcctcctctttttttgttttgttttgttttgtttttgttttgtttttttgagtcagggtctcccttgttgcccagactggagtgcattgatatgatcatagctcactgcagcctcggactcctgggctcaagccatcctcccactagccttccaagtaggtgagactacagctgcgtgccaccatgtctggctaatttttaaatttttagtagagatggggtctcgatatgttgcccagcaaatcctgggctcaagcgatcctcccgcctcagcctcccaaatcgctgggattacaggtgtgagccactgcacccagcctctcctcctcttataagaacacagtcatactggattaagggcttgccctaatgacctcaccttagtttcatagttacatctgcaaagaccctttttccaaataagtctgcattcacaggtattggggcttaggactttaacgtatcttttggtgggggatacagtacaacccacagcattttcataactcatattttcccttaacagacaatctttagagcatcgttggactgtgcctaaactgcaaattcttggaatcaccctgctggtgctggccttgtcacaaagcacagcctgggaaaggagcattccagaagagtatgtcagtgaacccaccagggggcactatgtgaccagaaaataaccccaaaacaccagcggttgcattaaattccattctgttaatgaatattgtttcttaactttatttcttaaatcagcaacttcacatttgataaagagtcaaggatttcctgatactcgaatcacagatttctgagcagctttaaaactcattgttcccctatatgtagcagtggattgctagtagccctaccaggtccttgaattgctctggaatgccaggtggagctaaattgaggggtcaggaactcctcattggatgtgagattcaagtgagaccatatatctaaaaataagttgaagagcaggatagccaatctctgcaggattggggtcaatctatctctgggaagtaatgttcaactctaagcaaagctgcacaagaagagaaatctgcattcggcactgcttcctggctggccccactgctcctcccttccttcctgttcagacacatgtcccacaaacttgcccccaaaccccattgcctaccaggtcccaaagaggccccaagttccaaagccacttcccccacaagcacaatttccagtttccttaaagtcagcagtaaggaaaggcctctccttaactgaaacaaaacgtgaaattcttttgggcaaatcaagaagggatctggaaggaaaacccacagggcagcctcagtatcagcagtccctgagtcccgcccctgggtggtgaatctgttccttgggattctggcatttcgccttaacacagaaggcgctcttctgggctgattaaaaggctcggcatattctctccatggttatccttactgtgtgcttataggtggtgccagcactcattcattcattccacagatgtttgttgggcacctaaaatgtgcctgacactgggacagatgctcagcgcacaccgccagagcgcccagcccgcgcacgtgcttccggcgcgcgccgaagtcctcacgcgccccgccccggcctccccgtgcgcacgcgcgaacgcggggtgggccgggcctcgcgtagcccatctcctcttcctcctcgcggtcgcggccggacggagggtggagggccc

SEQ ID NO: 15579 - RNA, 4023 nt, Homo sapiens
  source 1..4023: mol_type = other RNA
gctgggattacaggcatgagccactgtgcccagccagagcctagcttgtaatcactccgctctactacctcccaccttcctttctttgtgtaataagattgcagtacacagtgctgtacaataaacaaaatatttttatacacatagtcacacttcatcctcacagggatcctgaggcaggagaacagttacttttgtatttctccattttgcagtttataaaactgaggctcagaaaaattgaacttctttgcccaaggtcattcaggtactaagtggtagctgggactcaaagcagttcttccaactcaaatccccatttctttctgtattcgtctgcttgggctgccatcacaaagcagcataaaccgggaggcttaagcaacaaacatatctcatctcacagttctggacgctgaagtccaaaatcaaggcatcagcaggattagaactttctgaggggttgagagagactctattccatgtcccgctcctggcttctgggggctgctggcaatccttgcgcattcctcggtctgcaggtgcatcagtccagtgtctgtctccattgtcacatggcattctctccttgtgtgtctctctcctcctctttttttgttttgttttgttttgtttttgttttgtttttttgagtcagggtctcccttgttgcccagactggagtgcattgatatgatcatagctcactgcagcctcggactcctgggctcaagccatcctcccactagccttccaagtaggtgagactacagctgcgtgccaccatgtctggctaatttttaaatttttagtagagatggggtctcgatatgttgcccagcaaatcctgggctcaagcgatcctcccgcctcagcctcccaaatcgctgggattacaggtgtgagccactgcacccagcctctcctcctcttataagaacacagtcatactggattaagggcttgccctaatgacctcaccttagtttcatagttacatctgcaaagaccctttttccaaataagtctgcattcacaggtattggggcttaggactttaacgtatcttttggtgggggatacagtacaacccacagcattttcataactcatattttcccttaacagacaatctttagagcatcgttggactgtgcctaaactgcaaattcttggaatcaccctgctggtgctggccttgtcacaaagcacagcctgggaaaggagcattccagaagagtatgtcagtgaacccaccagggggcactatgtgaccagaaaataaccccaaaacaccagcggttgcattaaattccattctgttaatgaatattgtttcttaactttatttcttaaatcagcaacttcacatttgataaagagtcaaggatttcctgatactcgaatcacagatttctgagcagctttaaaactcattgttcccctatatgtagcagtggattgctagtagccctaccaggtccttgaattgctctggaatgccaggtggagctaaattgaggggtcaggaactcctcattggatgtgagattcaagtgagaccatatatctaaaaataagttgaagagcaggatagccaatctctgcaggattggggtcaatctatctctgggaagtaatgttcaactctaagcaaagctgcacaagaagagaaatctgcattcggcactgcttcctggctggccccactgctcctcccttccttcctgttcagacacatgtcccacaaacttgcccccaaaccccattgcctaccaggtcccaaagaggccccaagttccaaagccacttcccccacaagcacaatttccagtttccttaaagtcagcagtaaggaaaggcctctccttaactgaaacaaaacgtgaaattcttttgggcaaatcaagaagggatctggaaggaaaacccacagggcagcctcagtatcagcagtccctgagtcccgcccctgggtggtgaatctgttccttgggattctggcatttcgccttaacacagaaggcgctcttctgggctgattaaaaggctcggcatattctctccatggttatccttactgtgtgcttataggtggtgccagcactcattcattcattccacagatgtttgttgggcacctaaaatgtgcctgacactgggacagatggtatgtgcagttatgcctatacttcaataaaattgtttcaaataaaagcacgatgagctgcctggacaggtgaaaattccagtggtagtcataatgtctttccatagactttctcttctcctttctttcagggacataacaatattgcatttcctgtcctctttgaaattaagtgttgccacatgacttgctttggcccatgaaatgtaaatagaagttcttatagcaattcctggtaagtgcttctctaactaatgcacaatcagtcctaatgcatagccactcctacctgagtgattgtggagatgcatttagataaaacacactcggtcagcctgggtctaggagggcccatgagcaagtctctgctcgtgggagtggacaggtagtctgagcgaggaactttgctgcgtaagtcataaatgggttgagagatctgcattactgcagttaatctagcccattctgactgaatattccctagcaacagaggtatctgatcatggacatagttttgacagtggaaggtaaagtggcccagtgacctctgaggtgtctactttcttgaagatgtgagttatatgtcatagtctccaccagcctgggtgtggaattgagcttccattttcaagtctccacttgtatgtctggaatttggctccttctcaaggtaacacccagggattgctgagttcccaagtgctcagacacaagtccactcattttcttcaattccagttaccaaagaaagtcaccattccaccgaggctgtgaccagtgccctccaccaggcctagctccaagaatctcatgcatcaagccccagggctcctcacgttgggcattaaatgtaaggtcatgccacattctttaacattgtcaggaagcaggaaggaaagtaccagatacttgaaggacccactgacctggaaaaaagtgggatctagtttcagcttgaaaaaatccttcttcataattacatttcccttaggcaaatctctaacatgcctaggcttttgtatatctgtttttactgcgtcacaaacctcccccaaagagaagggagacgataactggagaaaaccacaaattaatcttccaatatttttttcttccatataatcagcagtgcctcagaatcaaagcagtctctaaaaatattttgaagaaatttattttcttggatcttcaaagatccaaagttactgagatgcaaagaatcttccacagtatcatccaaggatactgaagggctccttcaaacctcgcccttgtatatttcttcttccagttgtgatactgcagttacatttgcaaaccaaatgatccctttgggtggtttttccaaaacaaatcgtctttcccaaaggcctacctaagtcttcattttccacaaagtagaaaactgcccacagctttgaaatggcagcataatttgtatttctaccaccttgtccaggtttcagggatctctggtccagtttcagtcaataatgctaactatcactgcagctcactgacttctttcttgtacatagcagtttttcgcaggaagaaaacaaatctaacgaataggaataacttcaggtgatgctgttttcttcccgcttcctgggatcactgtctttcctctgaaatggttttaatcagaaccaatctgttatactcaggagcctcagcgcacaccgccagagcgcccagcccgcgcacgtgcttccggcgcgcgccgaagtcctcacgcgccccgccccggcctccccgtgcgcacgcgcgaacgcggggtgggccgggcctcgcgtagcccatctcctcttcctcctcgcggtcgcggccggacggagggtggagggccc

SEQ ID NO: 15580 - RNA, 1668 nt, Homo sapiens
  source 1..1668: mol_type = other RNA
gctgggattacaggcatgagccactgtgcccagccagctgtgaattttgacatgctgaattccataaagcctcaacagaaccactggaaatttctgtagaattgatctcttctgacctgcaacaagaggaatatcagagaaatgcaatttggccaatctaaagactccttccatattattaatctaacacaacactttagaaagatattttattttttaggaaaagagccataattatcttaaatgtgaaaaaccacatccaataaactgatataaagttttaggaacaagggaatatcttattgtcacgcattcacagtgaaacccattttaatgcaggtccagagccaactgcagtcctgtccaatcccataggtacaagggcctggctcctcttcctgtgtactgcccgacttcctcatcttactgggtccagcataaagcagatgtccactgtcttcctcacatgctgtgatcttggcttagaggtaggcacagtgccgctccagcagcgaggggttcgcgttacttaggaacagcagctcttttttcccttcttctgtaggagctttctcatgttgaagccaattgttttccaaataatactgaatacaactttcaaattcctttgggttatagttggaaaccaggatgggaataaagggatccagggcatcaaatccttcctttcccagcaactcctggggcagataggctttccggggcttaaagagagacccagtctggctcaaagccgacacaatggcgcctccatgccaatcatttttcatcattttcctcaagttgtgaacaagtgctaattcctcgggggcaatcgggcttttatcttctcttttcagagtggttcttccccaaagagcattgattccatccacggccactaggaggtgaaacatacccaaagaactttgcctctttagctctttcagcacaattccaactgcatctgtggcgttcctcacccgtgttatgccctgttcaaccacttctcccagaggactccctttctcagtgctttctctcttattccagacatacttctcttgaacttttatctggttcaggaagcgctcatttgtagttttgaaattcttcagccaggttgaagcctctaaaggttgatcaaagcgctgtttgttgtagctggactgcagaagatcccgacaatttttcacccaaagatgagcatctggaatatgtagtatcagccagtcctgttttgcacagaaatgaataacatggcaaagacttagggtttttcctgttcccttctctccatacagaagatatcgtatagctggataagcaaaactggtgtttttcaggtaatgcagaagttctagggctggtttccttaccatcaggcaagcttcactgaatgtcttcaccgggtcattctcattggtgcgggaaatagctctcggactctcaactggaacctggttatctaggtgagcagcaatgctttggcgagcctgggtccccatgtgtaaaaaacgcccagggtccaacttatggatcctagagataagccttgttattcctttcagcatcatccttgcacgtgagtcgaggactagttctccagactaggcgaccgacacacgctgcctggggccggctccaaagcgcccgtcctgagactgc

SEQ ID NO: 15581 - RNA, 1770 nt, Homo sapiens
  source 1..1770: mol_type = other RNA
gctgggattacaggcatgagccactgtgcccagccagctgtgaattttgacatgctgaattccataaagcctcaacagaaccactggaaatttctgtagaattgatctcttctgacctgcaacaagaggaatatcagagaaatgcaatttggccaatctaaagactccttccatattattaatctaacacaacactttagaaagatattttattttttaggaaaagagccataattatcttaaatgtgaaaaaccacatccaataaactgatataaagttttaggaacaagggaatatcttattgtcacgcattcacagtgaaacccattttaatgcaggtccagagccaactgcagtcctgtccaatcccataggtacaagggcctggctcctcttcctgtgtactgcccgacttcctcatcttactgggtccagcataaagcagatgtccactgtcttcctcacatgctgtgatcttggcttagaggtaggcacagtgccgctccagcagcgaggggttcgcgttacttaggaacagcagctcttttttcccttcttctgtaggagctttctcatgttgaagccaattgttttccaaataatactgaatacaactttcaaattcctttgggttatagttggaaaccaggatgggaataaagggatccagggcatcaaatccttcctttcccagcaactcctggggcagataggctttccggggcttaaagagagacccagtctggctcaaagccgacacaatggcgcctccatgccaatcatttttcatcattttcctcaagttgtgaacaagtgctaattcctcgggggcaatcgggcttttatcttctcttttcagagtggttcttccccaaagagcattgattccatccacggccactaggaggtgaaacatacccaaagaactttgcctctttagctctttcagcacaattccaactgcatctgtggcgttcctcacccgtgttatgccctgttcaaccacttctcccagaggactccctttctcagtgctttctctcttattccagacatacttctcttgaacttttatctggttcaggaagcgctcatttgtagttttgaaattcttcagccaggttgaagcctctaaaggttgatcaaagcgctgtttgttgtagctggactgcagaagatcccgacaatttttcacccaaagatgagcatctggaatatgtagtatcagccagtcctgttttgcacagaaatgaataacatggcaaagacttagggtttttcctgttcccttctctccatacagaagatatcgtatagctggataagcaaaactggtgtttttcaggtaatgcagaagttctagggctggtttccttaccatcaggcaagcttcactgaatgtcttcacctgcatcacaaagcgaggaggaaggccatggggaaatacagtctccaaatcctggggggagatgttgtagtgctgaccctcgtgctgatccccatgcttggccgggtcattctcattggtgcgggaaatagctctcggactctcaactggaacctggttatctaggtgagcagcaatgctttggcgagcctgggtccccatgtgtaaaaaacgcccagggtccaacttatggatcctagagataagccttgttattcctttcagcatcatccttgcacgtgagtcgaggactagttctccagactaggcgaccgacacacgctgcctggggccggctccaaagcgcccgtcctgagactgc

SEQ ID NO: 15582 - RNA, 1836 nt, Homo sapiens
  source 1..1836: mol_type = other RNA
gctgggattacaggcatgagccactgtgcccagccagctgtgaattttgacatgctgaattccataaagcctcaacagaaccactggaaatttctgtagaattgatctcttctgacctgcaacaagaggaatatcagagaaatgcaatttggccaatctaaagactccttccatattattaatctaacacaacactttagaaagatattttattttttaggaaaagagccataattatcttaaatgtgaaaaaccacatccaataaactgatataaagttttaggaacaagggaatatcttattgtcacgcattcacagtgaaacccattttaatgcaggtccagagccaactgcagtcctgtccaatcccataggtacaagggcctggctcctcttcctgtgtactgcccgacttcctcatcttactgggtccagcataaagcagatgtccactgtcttcctcacatgctgtgatcttggcttagaggtaggcacagtgccgctccagcagcgaggggttcgcgttacttaggaacagcagctcttttttcccttcttctgtaggagctttctcatgttgaagccaattgttttccaaataatactgaatacaactttcaaattcctttgggttatagttggaaaccaggatgggaataaagggatccagggcatcaaatccttcctttcccagcaactcctggggcagataggctttccggggcttaaagagagacccagtctggctcaaagccgacacaatggcgcctccatgccaatcatttttcatcattttcctcaagttgtgaacaagtgctaattcctcgggggcaatcgggcttttatcttctcttttcagagtggttcttccccaaagagcattgattccatccacggccactaggaggtgaaacatacccaaagaactttgcctctttagctctttcagcacaattccaactgcatctgtggcgttcctcacccgtgttatgccctgttcaaccacttctcccagaggactccctttctcagtgctttctctcttattccagacatacttctcttgaacttttatctggttcaggaagcgctcatttgtagttttgaaattcttcagccaggttgaagcctctaaaggttgatcaaagcgctgtttgttgtagctggactgcagaagatcccgacaatttttcacccaaagatgagcatctggaatatgtagtatcagccagtcctgttttgcacagaaatgaataacatggcaaagacttagggtttttcctgttcccttctctccatacagaagatatcgtatagctggataagcaaaactggtgtttttcaggtaatgcagaagttctagggctggtttccttaccatcaggcaagcttcactgaatgtcttcacctgcatcacaaagcgaggaggaaggccatggggaaatacagtctccaaatcctggggggagatgttgtagtgctgaccctcgtgctgatccccatgcttggccgggtcattctcattggtgcgggaaatagctctcggactctcaactggaacctggttatctaggtgagcagcaatgctttggcgagcctgggtccccatgtgtaaaaaacgcccagggtccaacttatggatcctagagataagccttgttattcctttcagcatcatccttgcactcctggaggtccggagtcccgctcctttccctcagcggtacaatacccgtgtcggtccattccctcaccgtgagtcgaggactagttctccagactaggcgaccgacacacgctgcctggggccggctccaaagcgcccgtcctgagac

SEQ ID NO: 15583 - RNA, 1863 nt, Homo sapiens
  source 1..1863: mol_type = other RNA
gctgggattacaggcatgagccactgtgcccagccagctgtgaattttgacatgctgaattccataaagcctcaacagaaccactggaaatttctgtagaattgatctcttctgacctgcaacaagaggaatatcagagaaatgcaatttggccaatctaaagactccttccatattattaatctaacacaacactttagaaagatattttattttttaggaaaagagccataattatcttaaatgtgaaaaaccacatccaataaactgatataaagttttaggaacaagggaatatcttattgtcacgcattcacagtgaaacccattttaatgcaggtccagagccaactgcagtcctgtccaatcccataggtacaagggcctggctcctcttcctgtgtactgcccgacttcctcatcttactgggtccagcataaagcagatgtccactgtcttcctcacatgctgtgatcttggcttagaggtaggcacagtgccgctccagcagcgaggggttcgcgttacttaggaacagcagctcttttttcccttcttctgtaggagctttctcatgttgaagccaattgttttccaaataatactgaatacaactttcaaattcctttgggttatagttggaaaccaggatgggaataaagggatccagggcatcaaatccttcctttcccagcaactcctggggcagataggctttccggggcttaaagagagacccagtctggctcaaagccgacacaatggcgcctccatgccaatcatttttcatcattttcctcaagttgtgaacaagtgctaattcctcgggggcaatcgggcttttatcttctcttttcagagtggttcttccccaaagagcattgattccatccacggccactaggaggtgaaacatacccaaagaactttgcctctttagctctttcagcacaattccaactgcatctgtggcgttcctcacccgtgttatgccctgttcaaccacttctcccagaggactccctttctcagtgctttctctcttattccagacatacttctcttgaacttttatctggttcaggaagcgctcatttgtagttttgaaattcttcagccaggttgaagcctctaaaggttgatcaaagcgctgtttgttgtagctggactgcagaagatcccgacaatttttcacccaaagatgagcatctggaatatgtagtatcagccagtcctgttttgcacagaaatgaataacatggcaaagacttagggtttttcctgttcccttctctccatacagaagatatcgtatagctggataagcaaaactggtgtttttcaggtaatgcagaagttctagggctggtttccttaccatcaggcaagcttcactgaatgtcttcacctgcatcacaaagcgaggaggaaggccatggggaaatacagtctccaaatcctggggggagatgttgtagtgctgaccctcgtgctgatccccatgcttggccgggtcattctcattggtgcgggaaatagctctcggactctcaactggaacctggttatctaggtgagcagcaatgctttggcgagcctgggtccccatgtgtaaaaaacgcccagggtccaacttatggatcctagagataagccttgttattcctttcagcatcatccttgcactgtaatcccagcactttgggaggtcaaggtgggcagatcacttgaggtcaggaattcgagaccagcctggccaacatggtaaaacttcatctcgtgagtcgaggactagttctccagactaggcgaccgacacacgctgcctggggccggctccaaagcgcccgtcctgagactgc

SEQ ID NO: 15584 - RNA, 1647 nt, Homo sapiens
  source 1..1647: mol_type = other RNA
gctgggattacaggcatgagccactgtgcccagccagctgtgaattttgacatgctgaattccataaagcctcaacagaaccactggaaatttctgtagaattgatctcttctgacctgcaacaagaggaatatcagagaaatgcaatttggccaatctaaagactccttccatattattaatctaacacaacactttagaaagatattttattttttaggaaaagagccataattatcttaaatgtgaaaaaccacatccaataaactgatataaagttttaggaacaagggaatatcttattgtcacgcattcacagtgaaacccattttaatgcaggtccagagccaactgcagtcctgtccaatcccataggtacaagggcctggctcctcttcctgtgtactgcccgacttcctcatcttactgggtccagcataaagcagatgtccactgtcttcctcacatgctgtgatcttggcttagaggtaggcacagtgccgctccagcagcgaggggttcgcgttacttaggaacagcagctcttttttcccttcttctgtaggagctttctcatgttgaagccaattgttttccaaataatactgaatacaactttcaaattcctttgggttatagttggaaaccaggatgggaataaagggatccagggcatcaaatccttcctttcccagcaactcctggggcagataggctttccggggcttaaagagagacccagtctggctcaaagccgacacaatggcgcctccatgccaatcatttttcatcattttcctcaagttgtgaacaagtgctaattcctcgggggcaatcgggcttttatcttctcttttcagagtggttcttccccaaagagcattgattccatccacggccactaggaggtgaaacatacccaaagaactttgcctctttagctctttcagcacaattccaactgcatctgtggcgttcctcacccgtgttatgccctgttcaaccacttctcccagaggactccctttctcagtgctttctctcttattccagacatacttctcttgaacttttatctggttcaggaagcgctcatttgtagttttgaaattcttcagccaggttgaagcctctaaaggttgatcaaagcgctgtttgttgtagctggactgcagaagatcccgacaatttttcacccaaagatgagcatctggaatatgtagtatcagccagtcctgttttgcacagaaatgaataacatggcaaagacttagggtttttcctgttcccttctctccatacagaagatatcgtatagctggataagcaaaactggtgtttttcaggtaatgcagaagttctagggctggtttccttaccatcaggcaagcttcactgaatgtcttcacctgcatcacaaagcgaggaggaaggccatggggaaatacagtctccaaatcctggggggagatgttgtagtgctgaccctcgtgctgatccccatgcttggccttatggatcctagagataagccttgttattcctttcagcatcatccttgcacgtgagtcgaggactagttctccagactaggcgaccgacacacgctgcctggggccggctccaaagcgcccgtcctgagactgc

SEQ ID NO: 15585 - RNA, 4724 nt, Homo sapiens
  source 1..4724: mol_type = other RNA
gctgggattacaggcatgagccactgtgcccagccaggaagttcatacacttgagtatgaacaaaaagttggaaaattaaatgctttaaaattacagcatggaaagacagaattatttggctgttgaactggtattctggtttagaaaattattcatttatttaaaattccaactttcccaaaatgttgcaaaatcaataattaaaggagaaaatattgtttaaggtaaaggtgcaaaataccatactgatacaacaatttgaacataaaaggagaagtcttgagtttttctaagtttgcaatcaagctcaatattggacttttctaaatttcatcagcatacaaaaaatattaactttgccaagcaacattattgagagaacattacaaaatccttacttagctaagggatggttcatgcatttttatggaaatatataatggtaagttctcaatgtgaagttttccatggggataatgcaactagtgaaacaaagtcaaatacatttcaaatgataaaatggaaatcttgtttccttatacagatagttcctgacttaagaggatgtgacttacagtttctcaacattacaatggtatccatacactactatttttcaccttcagtattcaataattacatcagatattcaacacctttttataaaatagatgatgcattagaatgtgttctgagaatgtttaaggtaggctacgctaagctatgatgtttggtaagttgggtgtattaaatgcatttttgacttacaatgttttcaacttacaatgggtttattgggaggtaaccccactgtaagtccaggatcatctgtacttttccagggaccacagaaatttgctagaagataaaataggcatccttgaatgtcaaaaatgtttttccagcacaaaattccctaatactttacatcttcagaaatgtgattttttaataattcatttatccatctaatttttacaagatattttatgcaacacaaaaagcataacagcagcacaaaatatccatgatactttatcacagtaaattaaaatagtgacatttgggttacatatcacttaagatacatatatatatactatatggaggcacctcactaaatgagaaaaagatttaatacagcactactttatttcatttagtttgggtgttgtaatgtagttcacacacctttattttgctcattcagttatatattactatggttattctgtggttcctgcctttgcatatttattttatataaactgttactcagactctgaggatgcagaagacttacacaatgttggcttcagttactgaatagaaaggtccataaaaacaaaagaccccttatgtatgtctataagttaaaagaaacgggttatcacttaaggtacttattcatgtagtcatgttacatgagtttccattttttatattattgttaaaaaataaaaaccagtggtgtgtagtgttgtcttcacagacatcagaggcactaaaaggcatatgcatttcatactcccaattacattaaattataggtaagtccaaaacacaaaacatacgtgacactagaagataagccacaaataccactaagaaatgtcttagatgtttcaataaccaatttattcacgtatttttaaaacttcacacttcaaagtgaacatctgtcaaccacttagaattgggtatttttggtacccatgtctacaaaaagtgtatggcttcccttgacagtactatactgaggggcaagtgttcccagtgtctttaaattgttaggttctccataatatgaattctccaaaatacaaaatagtctcgttacttgttgcactgtcccatatttagtactttcatagaacttcattcctaagagcattttcttatgtacaatgaactgtcatttcttaaaaatattgcctcatttcccgcattcatggggttttccctcatccccagtgggaatatttctaatagcttaagagacttgacttctggaaggcttttggacattcacaggattcttctttgctgtgaatgttctactctataaggcttgtctatggttttaaaagtttttgagatccactgcagtcataggttcactctactctatgaattatgatcggctttccatacaccacctcatttagagttctcatcctcatggagtacaaacacctaacatgacgtgactgtctacaaacgttatcataattgcatttcctgaagtccaagatgatctgtcaaagactactattaactgtattcctaggatttttttactgtatgagttctctgatgattgatgagctgtgacttctgtgagaaagctttcccacattcaatgcatcgataaggcttctctcctgtatgaattctctgatgattaaccagctgtgacttctgagagaaggccttcctacattcactgcatccatagggtttctcacccgtatgtgtcctttgatgtggtataaggtgtgacttccgagagaaagctttgccacactcactgcattcaaaaggcttctctcctgtatgtattctctgatgattgatgagacttgacttctccctgaaggcttttctacattcattgcattcataaggtttttctcctgtatgagttctcagatgtctaattagctccgacttctcaaaaaaagctttcctacaaagactgcattcatagggtttctctccagtgtgaattctctgatgggtatttagctgtgatttctgggagaaagctttttcacagtccctgcattcatacggtttttctccagtatgagttctctgatgagttgcaagacttgacttctcaccaaaggccttcccacattcactgcattcatagggtttctcccctgtatgtgtcctctgatgtgatatgagatgtgacttctgacaaaaggctttcccacattcactgcatacatatggtttttctcctgtatgaattctttgatgattagtgagacttaatttttcactgaaagctttcccacactcactgcattcatacggtttttctcccgtatgagttctctgatgtctaacgagctgtgatttcctgctgaaggctttcccacatttactgcatataaagggtttttctcctgtgtgtgtcatctgatgtgatatgagatgtgacttctgggagaaggccttcccacactgaatgcatccatgaggtttctctcctgtatgtgttctctgatgattaatgagactcgacctctctctaaatgctttcctacactcgctgcattcatagggtttctctccagtatgaattgtctgatgtctaataagctctgacttctcaaagaatgcttttctacaatcactacatccaaagggttttgttcctgtgtgagttctgtgatgtgtaacgagttgtgacttcctgctgaaggctttcccacattccctgcattcaaaaggcttctcaccggtatgaattctctgatggttaatgagattggacttttcactaaaggccctcccacattcattgcatccatagggtttctctcctgtgtgtgttctccaatgcgatatgagatgtgacttccgggagaaggctttcccacattcaccacactcataaggtttctctcctgtatgtgtccgctgatgggatgtgagctgtgacttttgggagaaggctttcccacactggctacaattataaggtttttctcctgtatgagttctgtgatgtgtaataaactgagacttctggggaaaggttttgccacaattaccacagccaaaggctatgtctcttatatgtctgctctgatgtttaatgagacttggtttcttactgaagcgcttcctacattcactgcattcatagagtttctcccctaaacgatttctatgatatatgataatctgtgactttttatagctctctttatatttatcacagtcatagtattttaaccaggtatcagtatcctcaggcttggaatggagaaaaaaattatcaaacacattaaagtcatctgattctgcttttccataatctccttttggaataagcaaatctaaatgatgttttaaaatcaatccatctaagtcaccttcactgtttgatttccttaaaggaacaaagttcatgttcagattgaaattttttccaaatgcatcacattcatgacctctttttataattttaagcttgtcttggttatcctggtgccacatcatgttaccatctactttccagacttctggagaatctgaacttggaatttctccatctcctacccacggctcttctccttgctccaatttgaagatgacatctggtttcataacttcataccccagtgacactaggctgctatagttctccaacatcacatccttgtataaattcttctgagagggatccagtagctgccactccttttgggtgaagtccacagataaatcgtcaaatgagaatgactcctgtaacatggtcattttctgctgctgtacgagatgatcagcaaggctgagatcggttctactgtgcgtctcttctgcttctgccccaaaactgtggagtgaggtctcagctaggtcttctacactgagaatgaattcctggttccaggaactcctttcttatctcacatgagcaggcttatttgtagggaccaggataaaagacgccgccgccgagtcgcgcccgcgcgcccgc

SEQ ID NO: 15586 - RNA, 4731 nt, Homo sapiens
  source 1..4731: mol_type = other RNA
gctgggattacaggcatgagccactgtgcccagccaggaagttcatacacttgagtatgaacaaaaagttggaaaattaaatgctttaaaattacagcatggaaagacagaattatttggctgttgaactggtattctggtttagaaaattattcatttatttaaaattccaactttcccaaaatgttgcaaaatcaataattaaaggagaaaatattgtttaaggtaaaggtgcaaaataccatactgatacaacaatttgaacataaaaggagaagtcttgagtttttctaagtttgcaatcaagctcaatattggacttttctaaatttcatcagcatacaaaaaatattaactttgccaagcaacattattgagagaacattacaaaatccttacttagctaagggatggttcatgcatttttatggaaatatataatggtaagttctcaatgtgaagttttccatggggataatgcaactagtgaaacaaagtcaaatacatttcaaatgataaaatggaaatcttgtttccttatacagatagttcctgacttaagaggatgtgacttacagtttctcaacattacaatggtatccatacactactatttttcaccttcagtattcaataattacatcagatattcaacacctttttataaaatagatgatgcattagaatgtgttctgagaatgtttaaggtaggctacgctaagctatgatgtttggtaagttgggtgtattaaatgcatttttgacttacaatgttttcaacttacaatgggtttattgggaggtaaccccactgtaagtccaggatcatctgtacttttccagggaccacagaaatttgctagaagataaaataggcatccttgaatgtcaaaaatgtttttccagcacaaaattccctaatactttacatcttcagaaatgtgattttttaataattcatttatccatctaatttttacaagatattttatgcaacacaaaaagcataacagcagcacaaaatatccatgatactttatcacagtaaattaaaatagtgacatttgggttacatatcacttaagatacatatatatatactatatggaggcacctcactaaatgagaaaaagatttaatacagcactactttatttcatttagtttgggtgttgtaatgtagttcacacacctttattttgctcattcagttatatattactatggttattctgtggttcctgcctttgcatatttattttatataaactgttactcagactctgaggatgcagaagacttacacaatgttggcttcagttactgaatagaaaggtccataaaaacaaaagaccccttatgtatgtctataagttaaaagaaacgggttatcacttaaggtacttattcatgtagtcatgttacatgagtttccattttttatattattgttaaaaaataaaaaccagtggtgtgtagtgttgtcttcacagacatcagaggcactaaaaggcatatgcatttcatactcccaattacattaaattataggtaagtccaaaacacaaaacatacgtgacactagaagataagccacaaataccactaagaaatgtcttagatgtttcaataaccaatttattcacgtatttttaaaacttcacacttcaaagtgaacatctgtcaaccacttagaattgggtatttttggtacccatgtctacaaaaagtgtatggcttcccttgacagtactatactgaggggcaagtgttcccagtgtctttaaattgttaggttctccataatatgaattctccaaaatacaaaatagtctcgttacttgttgcactgtcccatatttagtactttcatagaacttcattcctaagagcattttcttatgtacaatgaactgtcatttcttaaaaatattgcctcatttcccgcattcatggggttttccctcatccccagtgggaatatttctaatagcttaagagacttgacttctggaaggcttttggacattcacaggattcttctttgctgtgaatgttctactctataaggcttgtctatggttttaaaagtttttgagatccactgcagtcataggttcactctactctatgaattatgatcggctttccatacaccacctcatttagagttctcatcctcatggagtacaaacacctaacatgacgtgactgtctacaaacgttatcataattgcatttcctgaagtccaagatgatctgtcaaagactactattaactgtattcctaggatttttttactgtatgagttctctgatgattgatgagctgtgacttctgtgagaaagctttcccacattcaatgcatcgataaggcttctctcctgtatgaattctctgatgattaaccagctgtgacttctgagagaaggccttcctacattcactgcatccatagggtttctcacccgtatgtgtcctttgatgtggtataaggtgtgacttccgagagaaagctttgccacactcactgcattcaaaaggcttctctcctgtatgtattctctgatgattgatgagacttgacttctccctgaaggcttttctacattcattgcattcataaggtttttctcctgtatgagttctcagatgtctaattagctccgacttctcaaaaaaagctttcctacaaagactgcattcatagggtttctctccagtgtgaattctctgatgggtatttagctgtgatttctgggagaaagctttttcacagtccctgcattcatacggtttttctccagtatgagttctctgatgagttgcaagacttgacttctcaccaaaggccttcccacattcactgcattcatagggtttctcccctgtatgtgtcctctgatgtgatatgagatgtgacttctgacaaaaggctttcccacattcactgcatacatatggtttttctcctgtatgaattctttgatgattagtgagacttaatttttcactgaaagctttcccacactcactgcattcatacggtttttctcccgtatgagttctctgatgtctaacgagctgtgatttcctgctgaaggctttcccacatttactgcatataaagggtttttctcctgtgtgtgtcatctgatgtgatatgagatgtgacttctgggagaaggccttcccacactgaatgcatccatgaggtttctctcctgtatgtgttctctgatgattaatgagactcgacctctctctaaatgctttcctacactcgctgcattcatagggtttctctccagtatgaattgtctgatgtctaataagctctgacttctcaaagaatgcttttctacaatcactacatccaaagggttttgttcctgtgtgagttctgtgatgtgtaacgagttgtgacttcctgctgaaggctttcccacattccctgcattcaaaaggcttctcaccggtatgaattctctgatggttaatgagattggacttttcactaaaggccctcccacattcattgcatccatagggtttctctcctgtgtgtgttctccaatgcgatatgagatgtgacttccgggagaaggctttcccacattcaccacactcataaggtttctctcctgtatgtgtccgctgatgggatgtgagctgtgacttttgggagaaggctttcccacactggctacaattataaggtttttctcctgtatgagttctgtgatgtgtaataaactgagacttctggggaaaggttttgccacaattaccacagccaaaggctatgtctcttatatgtctgctctgatgtttaatgagacttggtttcttactgaagcgcttcctacattcactgcattcatagagtttctcccctaaacgatttctatgatatatgataatctgtgactttttatagctctctttatatttatcacagtcatagtattttaaccaggtatcagtatcctcaggcttggaatggagaaaaaaattatcaaacacattaaagtcatctgattctgcttttccataatctccttttggaataagcaaatctaaatgatgttttaaaatcaatccatctaagtcaccttcactgtttgatttccttaaaggaacaaagttcatgttcagattgaaattttttccaaatgcatcacattcatgacctctttttataattttaagcttgtcttggttatcctggtgccacatcatgttaccatctactttccagacttctggagaatctgaacttggaatttctccatctcctacccacggctcttctccttgctccaatttgaagatgacatctggtttcataacttcataccccagtgacactaggctgctatagttctccaacatcacatccttgtataaattcttctgagagggatccagtagctgccactccttttgggtgaagtccacagataaatcgtcaaatgagaatgactcctgtaacatggtcattttctgctgctgtacgagatgatcagcaaggctgagatcggttctactgtgcgtctcttctgcttctgccccaaaactgtggagtgaggtctcagctaggtcttctacactgagaatgaattcctggttccaggaactcctttcttatctcacatgagcaggcttatttgtagggaccaggatctgtggaaaaagacgccgccgccgagtcgcgcccgcgcgcccgc

SEQ ID NO: 15587 - RNA, 4853 nt, Homo sapiens
  source 1..4853: mol_type = other RNA
gctgggattacaggcatgagccactgtgcccagccaggaagttcatacacttgagtatgaacaaaaagttggaaaattaaatgctttaaaattacagcatggaaagacagaattatttggctgttgaactggtattctggtttagaaaattattcatttatttaaaattccaactttcccaaaatgttgcaaaatcaataattaaaggagaaaatattgtttaaggtaaaggtgcaaaataccatactgatacaacaatttgaacataaaaggagaagtcttgagtttttctaagtttgcaatcaagctcaatattggacttttctaaatttcatcagcatacaaaaaatattaactttgccaagcaacattattgagagaacattacaaaatccttacttagctaagggatggttcatgcatttttatggaaatatataatggtaagttctcaatgtgaagttttccatggggataatgcaactagtgaaacaaagtcaaatacatttcaaatgataaaatggaaatcttgtttccttatacagatagttcctgacttaagaggatgtgacttacagtttctcaacattacaatggtatccatacactactatttttcaccttcagtattcaataattacatcagatattcaacacctttttataaaatagatgatgcattagaatgtgttctgagaatgtttaaggtaggctacgctaagctatgatgtttggtaagttgggtgtattaaatgcatttttgacttacaatgttttcaacttacaatgggtttattgggaggtaaccccactgtaagtccaggatcatctgtacttttccagggaccacagaaatttgctagaagataaaataggcatccttgaatgtcaaaaatgtttttccagcacaaaattccctaatactttacatcttcagaaatgtgattttttaataattcatttatccatctaatttttacaagatattttatgcaacacaaaaagcataacagcagcacaaaatatccatgatactttatcacagtaaattaaaatagtgacatttgggttacatatcacttaagatacatatatatatactatatggaggcacctcactaaatgagaaaaagatttaatacagcactactttatttcatttagtttgggtgttgtaatgtagttcacacacctttattttgctcattcagttatatattactatggttattctgtggttcctgcctttgcatatttattttatataaactgttactcagactctgaggatgcagaagacttacacaatgttggcttcagttactgaatagaaaggtccataaaaacaaaagaccccttatgtatgtctataagttaaaagaaacgggttatcacttaaggtacttattcatgtagtcatgttacatgagtttccattttttatattattgttaaaaaataaaaaccagtggtgtgtagtgttgtcttcacagacatcagaggcactaaaaggcatatgcatttcatactcccaattacattaaattataggtaagtccaaaacacaaaacatacgtgacactagaagataagccacaaataccactaagaaatgtcttagatgtttcaataaccaatttattcacgtatttttaaaacttcacacttcaaagtgaacatctgtcaaccacttagaattgggtatttttggtacccatgtctacaaaaagtgtatggcttcccttgacagtactatactgaggggcaagtgttcccagtgtctttaaattgttaggttctccataatatgaattctccaaaatacaaaatagtctcgttacttgttgcactgtcccatatttagtactttcatagaacttcattcctaagagcattttcttatgtacaatgaactgtcatttcttaaaaatattgcctcatttcccgcattcatggggttttccctcatccccagtgggaatatttctaatagcttaagagacttgacttctggaaggcttttggacattcacaggattcttctttgctgtgaatgttctactctataaggcttgtctatggttttaaaagtttttgagatccactgcagtcataggttcactctactctatgaattatgatcggctttccatacaccacctcatttagagttctcatcctcatggagtacaaacacctaacatgacgtgactgtctacaaacgttatcataattgcatttcctgaagtccaagatgatctgtcaaagactactattaactgtattcctaggatttttttactgtatgagttctctgatgattgatgagctgtgacttctgtgagaaagctttcccacattcaatgcatcgataaggcttctctcctgtatgaattctctgatgattaaccagctgtgacttctgagagaaggccttcctacattcactgcatccatagggtttctcacccgtatgtgtcctttgatgtggtataaggtgtgacttccgagagaaagctttgccacactcactgcattcaaaaggcttctctcctgtatgtattctctgatgattgatgagacttgacttctccctgaaggcttttctacattcattgcattcataaggtttttctcctgtatgagttctcagatgtctaattagctccgacttctcaaaaaaagctttcctacaaagactgcattcatagggtttctctccagtgtgaattctctgatgggtatttagctgtgatttctgggagaaagctttttcacagtccctgcattcatacggtttttctccagtatgagttctctgatgagttgcaagacttgacttctcaccaaaggccttcccacattcactgcattcatagggtttctcccctgtatgtgtcctctgatgtgatatgagatgtgacttctgacaaaaggctttcccacattcactgcatacatatggtttttctcctgtatgaattctttgatgattagtgagacttaatttttcactgaaagctttcccacactcactgcattcatacggtttttctcccgtatgagttctctgatgtctaacgagctgtgatttcctgctgaaggctttcccacatttactgcatataaagggtttttctcctgtgtgtgtcatctgatgtgatatgagatgtgacttctgggagaaggccttcccacactgaatgcatccatgaggtttctctcctgtatgtgttctctgatgattaatgagactcgacctctctctaaatgctttcctacactcgctgcattcatagggtttctctccagtatgaattgtctgatgtctaataagctctgacttctcaaagaatgcttttctacaatcactacatccaaagggttttgttcctgtgtgagttctgtgatgtgtaacgagttgtgacttcctgctgaaggctttcccacattccctgcattcaaaaggcttctcaccggtatgaattctctgatggttaatgagattggacttttcactaaaggccctcccacattcattgcatccatagggtttctctcctgtgtgtgttctccaatgcgatatgagatgtgacttccgggagaaggctttcccacattcaccacactcataaggtttctctcctgtatgtgtccgctgatgggatgtgagctgtgacttttgggagaaggctttcccacactggctacaattataaggtttttctcctgtatgagttctgtgatgtgtaataaactgagacttctggggaaaggttttgccacaattaccacagccaaaggctatgtctcttatatgtctgctctgatgtttaatgagacttggtttcttactgaagcgcttcctacattcactgcattcatagagtttctcccctaaacgatttctatgatatatgataatctgtgactttttatagctctctttatatttatcacagtcatagtattttaaccaggtatcagtatcctcaggcttggaatggagaaaaaaattatcaaacacattaaagtcatctgattctgcttttccataatctccttttggaataagcaaatctaaatgatgttttaaaatcaatccatctaagtcaccttcactgtttgatttccttaaaggaacaaagttcatgttcagattgaaattttttccaaatgcatcacattcatgacctctttttataattttaagcttgtcttggttatcctggtgccacatcatgttaccatctactttccagacttctggagaatctgaacttggaatttctccatctcctacccacggctcttctccttgctccaatttgaagatgacatctggtttcataacttcataccccagtgacactaggctgctatagttctccaacatcacatccttgtataaattcttctgagagggatccagtagctgccactccttttgggtgaagtccacagataaatcgtcaaatgagaatgactcctgtaacatggtcattttctgctgctgtacgagatgatcagcaaggctgagatcggttctactgtgcgtctcttctgcttctgccccaaaactgtggagtgaggtctcagctaggtcttctacactgagaatgaattcctggttccaggaactcctttcttatctcacatgagcaggcttatttgtagggaccaggatctgtggacacaggtaaccattcttaggatgatggaaactattgtgatatttttcatacaatggaagcatatggtcatatttaaaagctgtttttgtttttttcccattatgtgaagaacatctttccaggtcaataaccttatttaaaagacgccgccgccgagtc

SEQ ID NO: 15588 - RNA, 5084 nt, Homo sapiens
  source 1..5084: mol_type = other RNA
gctgggattacaggcatgagccactgtgcccagccaggaagttcatacacttgagtatgaacaaaaagttggaaaattaaatgctttaaaattacagcatggaaagacagaattatttggctgttgaactggtattctggtttagaaaattattcatttatttaaaattccaactttcccaaaatgttgcaaaatcaataattaaaggagaaaatattgtttaaggtaaaggtgcaaaataccatactgatacaacaatttgaacataaaaggagaagtcttgagtttttctaagtttgcaatcaagctcaatattggacttttctaaatttcatcagcatacaaaaaatattaactttgccaagcaacattattgagagaacattacaaaatccttacttagctaagggatggttcatgcatttttatggaaatatataatggtaagttctcaatgtgaagttttccatggggataatgcaactagtgaaacaaagtcaaatacatttcaaatgataaaatggaaatcttgtttccttatacagatagttcctgacttaagaggatgtgacttacagtttctcaacattacaatggtatccatacactactatttttcaccttcagtattcaataattacatcagatattcaacacctttttataaaatagatgatgcattagaatgtgttctgagaatgtttaaggtaggctacgctaagctatgatgtttggtaagttgggtgtattaaatgcatttttgacttacaatgttttcaacttacaatgggtttattgggaggtaaccccactgtaagtccaggatcatctgtacttttccagggaccacagaaatttgctagaagataaaataggcatccttgaatgtcaaaaatgtttttccagcacaaaattccctaatactttacatcttcagaaatgtgattttttaataattcatttatccatctaatttttacaagatattttatgcaacacaaaaagcataacagcagcacaaaatatccatgatactttatcacagtaaattaaaatagtgacatttgggttacatatcacttaagatacatatatatatactatatggaggcacctcactaaatgagaaaaagatttaatacagcactactttatttcatttagtttgggtgttgtaatgtagttcacacacctttattttgctcattcagttatatattactatggttattctgtggttcctgcctttgcatatttattttatataaactgttactcagactctgaggatgcagaagacttacacaatgttggcttcagttactgaatagaaaggtccataaaaacaaaagaccccttatgtatgtctataagttaaaagaaacgggttatcacttaaggtacttattcatgtagtcatgttacatgagtttccattttttatattattgttaaaaaataaaaaccagtggtgtgtagtgttgtcttcacagacatcagaggcactaaaaggcatatgcatttcatactcccaattacattaaattataggtaagtccaaaacacaaaacatacgtgacactagaagataagccacaaataccactaagaaatgtcttagatgtttcaataaccaatttattcacgtatttttaaaacttcacacttcaaagtgaacatctgtcaaccacttagaattgggtatttttggtacccatgtctacaaaaagtgtatggcttcccttgacagtactatactgaggggcaagtgttcccagtgtctttaaattgttaggttctccataatatgaattctccaaaatacaaaatagtctcgttacttgttgcactgtcccatatttagtactttcatagaacttcattcctaagagcattttcttatgtacaatgaactgtcatttcttaaaaatattgcctcatttcccgcattcatggggttttccctcatccccagtgggaatatttctaatagcttaagagacttgacttctggaaggcttttggacattcacaggattcttctttgctgtgaatgttctactctataaggcttgtctatggttttaaaagtttttgagatccactgcagtcataggttcactctactctatgaattatgatcggctttccatacaccacctcatttagagttctcatcctcatggagtacaaacacctaacatgacgtgactgtctacaaacgttatcataattgcatttcctgaagtccaagatgatctgtcaaagactactattaactgtattcctaggatttttttactgtatgagttctctgatgattgatgagctgtgacttctgtgagaaagctttcccacattcaatgcatcgataaggcttctctcctgtatgaattctctgatgattaaccagctgtgacttctgagagaaggccttcctacattcactgcatccatagggtttctcacccgtatgtgtcctttgatgtggtataaggtgtgacttccgagagaaagctttgccacactcactgcattcaaaaggcttctctcctgtatgtattctctgatgattgatgagacttgacttctccctgaaggcttttctacattcattgcattcataaggtttttctcctgtatgagttctcagatgtctaattagctccgacttctcaaaaaaagctttcctacaaagactgcattcatagggtttctctccagtgtgaattctctgatgggtatttagctgtgatttctgggagaaagctttttcacagtccctgcattcatacggtttttctccagtatgagttctctgatgagttgcaagacttgacttctcaccaaaggccttcccacattcactgcattcatagggtttctcccctgtatgtgtcctctgatgtgatatgagatgtgacttctgacaaaaggctttcccacattcactgcatacatatggtttttctcctgtatgaattctttgatgattagtgagacttaatttttcactgaaagctttcccacactcactgcattcatacggtttttctcccgtatgagttctctgatgtctaacgagctgtgatttcctgctgaaggctttcccacatttactgcatataaagggtttttctcctgtgtgtgtcatctgatgtgatatgagatgtgacttctgggagaaggccttcccacactgaatgcatccatgaggtttctctcctgtatgtgttctctgatgattaatgagactcgacctctctctaaatgctttcctacactcgctgcattcatagggtttctctccagtatgaattgtctgatgtctaataagctctgacttctcaaagaatgcttttctacaatcactacatccaaagggttttgttcctgtgtgagttctgtgatgtgtaacgagttgtgacttcctgctgaaggctttcccacattccctgcattcaaaaggcttctcaccggtatgaattctctgatggttaatgagattggacttttcactaaaggccctcccacattcattgcatccatagggtttctctcctgtgtgtgttctccaatgcgatatgagatgtgacttccgggagaaggctttcccacattcaccacactcataaggtttctctcctgtatgtgtccgctgatgggatgtgagctgtgacttttgggagaaggctttcccacactggctacaattataaggtttttctcctgtatgagttctgtgatgtgtaataaactgagacttctggggaaaggttttgccacaattaccacagccaaaggctatgtctcttatatgtctgctctgatgtttaatgagacttggtttcttactgaagcgcttcctacattcactgcattcatagagtttctcccctaaacgatttctatgatatatgataatctgtgactttttatagctctctttatatttatcacagtcatagtattttaaccaggtatcagtatcctcaggcttggaatggagaaaaaaattatcaaacacattaaagtcatctgattctgcttttccataatctccttttggaataagcaaatctaaatgatgttttaaaatcaatccatctaagtcaccttcactgtttgatttccttaaaggaacaaagttcatgttcagattgaaattttttccaaatgcatcacattcatgacctctttttataattttaagcttgtcttggttatcctggtgccacatcatgttaccatctactttccagacttctggagaatctgaacttggaatttctccatctcctacccacggctcttctccttgctccaatttgaagatgacatctggtttcataacttcataccccagtgacactaggctgctatagttctccaacatcacatccttgtataaattcttctgagagggatccagtagctgccactccttttgggtgaagtccacagataaatcgtcaaatgagaatgactcctgtaacatggtcattttctgctgctgtacgagatgatcagcaaggctgagatcggttctactgtgcgtctcttctgcttctgccccaaaactgtggagtgaggtctcagctaggtcttctacactgagaatgaattcctggttccaggaactcctttcttatctcacatgagcaggcttatttgtagggaccaggatctgtggactgtaaccccagcgctttaaaagcctccttcgatagcggcagagccaggctgctggtggatgcggtccagcagggcagccgctccttagggccacggcgcggcaagcgggctggcccgaggtcgaggctaaacgcgcccgaggctaaacgcgcccgaggctggcgcctccacgcccgcctgaaaggacgcccaggagcggcgcctccggaaaggccgtgcccgccccacagcccagaatccgcgcagctccgcggcccacggcatcttcacgacccggcccagccccaacccgccccagacccgcatccgcgcgcggacgcccagggccttgaagccgaagctccccgcggccactcccgcgcgcctcccccgccattcccggagccccc

SEQ ID NO: 15589 - RNA, 5117 nt, Homo sapiens
  source 1..5117: mol_type = other RNA
gctgggattacaggcatgagccactgtgcccagccaggaagttcatacacttgagtatgaacaaaaagttggaaaattaaatgctttaaaattacagcatggaaagacagaattatttggctgttgaactggtattctggtttagaaaattattcatttatttaaaattccaactttcccaaaatgttgcaaaatcaataattaaaggagaaaatattgtttaaggtaaaggtgcaaaataccatactgatacaacaatttgaacataaaaggagaagtcttgagtttttctaagtttgcaatcaagctcaatattggacttttctaaatttcatcagcatacaaaaaatattaactttgccaagcaacattattgagagaacattacaaaatccttacttagctaagggatggttcatgcatttttatggaaatatataatggtaagttctcaatgtgaagttttccatggggataatgcaactagtgaaacaaagtcaaatacatttcaaatgataaaatggaaatcttgtttccttatacagatagttcctgacttaagaggatgtgacttacagtttctcaacattacaatggtatccatacactactatttttcaccttcagtattcaataattacatcagatattcaacacctttttataaaatagatgatgcattagaatgtgttctgagaatgtttaaggtaggctacgctaagctatgatgtttggtaagttgggtgtattaaatgcatttttgacttacaatgttttcaacttacaatgggtttattgggaggtaaccccactgtaagtccaggatcatctgtacttttccagggaccacagaaatttgctagaagataaaataggcatccttgaatgtcaaaaatgtttttccagcacaaaattccctaatactttacatcttcagaaatgtgattttttaataattcatttatccatctaatttttacaagatattttatgcaacacaaaaagcataacagcagcacaaaatatccatgatactttatcacagtaaattaaaatagtgacatttgggttacatatcacttaagatacatatatatatactatatggaggcacctcactaaatgagaaaaagatttaatacagcactactttatttcatttagtttgggtgttgtaatgtagttcacacacctttattttgctcattcagttatatattactatggttattctgtggttcctgcctttgcatatttattttatataaactgttactcagactctgaggatgcagaagacttacacaatgttggcttcagttactgaatagaaaggtccataaaaacaaaagaccccttatgtatgtctataagttaaaagaaacgggttatcacttaaggtacttattcatgtagtcatgttacatgagtttccattttttatattattgttaaaaaataaaaaccagtggtgtgtagtgttgtcttcacagacatcagaggcactaaaaggcatatgcatttcatactcccaattacattaaattataggtaagtccaaaacacaaaacatacgtgacactagaagataagccacaaataccactaagaaatgtcttagatgtttcaataaccaatttattcacgtatttttaaaacttcacacttcaaagtgaacatctgtcaaccacttagaattgggtatttttggtacccatgtctacaaaaagtgtatggcttcccttgacagtactatactgaggggcaagtgttcccagtgtctttaaattgttaggttctccataatatgaattctccaaaatacaaaatagtctcgttacttgttgcactgtcccatatttagtactttcatagaacttcattcctaagagcattttcttatgtacaatgaactgtcatttcttaaaaatattgcctcatttcccgcattcatggggttttccctcatccccagtgggaatatttctaatagcttaagagacttgacttctggaaggcttttggacattcacaggattcttctttgctgtgaatgttctactctataaggcttgtctatggttttaaaagtttttgagatccactgcagtcataggttcactctactctatgaattatgatcggctttccatacaccacctcatttagagttctcatcctcatggagtacaaacacctaacatgacgtgactgtctacaaacgttatcataattgcatttcctgaagtccaagatgatctgtcaaagactactattaactgtattcctaggatttttttactgtatgagttctctgatgattgatgagctgtgacttctgtgagaaagctttcccacattcaatgcatcgataaggcttctctcctgtatgaattctctgatgattaaccagctgtgacttctgagagaaggccttcctacattcactgcatccatagggtttctcacccgtatgtgtcctttgatgtggtataaggtgtgacttccgagagaaagctttgccacactcactgcattcaaaaggcttctctcctgtatgtattctctgatgattgatgagacttgacttctccctgaaggcttttctacattcattgcattcataaggtttttctcctgtatgagttctcagatgtctaattagctccgacttctcaaaaaaagctttcctacaaagactgcattcatagggtttctctccagtgtgaattctctgatgggtatttagctgtgatttctgggagaaagctttttcacagtccctgcattcatacggtttttctccagtatgagttctctgatgagttgcaagacttgacttctcaccaaaggccttcccacattcactgcattcatagggtttctcccctgtatgtgtcctctgatgtgatatgagatgtgacttctgacaaaaggctttcccacattcactgcatacatatggtttttctcctgtatgaattctttgatgattagtgagacttaatttttcactgaaagctttcccacactcactgcattcatacggtttttctcccgtatgagttctctgatgtctaacgagctgtgatttcctgctgaaggctttcccacatttactgcatataaagggtttttctcctgtgtgtgtcatctgatgtgatatgagatgtgacttctgggagaaggccttcccacactgaatgcatccatgaggtttctctcctgtatgtgttctctgatgattaatgagactcgacctctctctaaatgctttcctacactcgctgcattcatagggtttctctccagtatgaattgtctgatgtctaataagctctgacttctcaaagaatgcttttctacaatcactacatccaaagggttttgttcctgtgtgagttctgtgatgtgtaacgagttgtgacttcctgctgaaggctttcccacattccctgcattcaaaaggcttctcaccggtatgaattctctgatggttaatgagattggacttttcactaaaggccctcccacattcattgcatccatagggtttctctcctgtgtgtgttctccaatgcgatatgagatgtgacttccgggagaaggctttcccacattcaccacactcataaggtttctctcctgtatgtgtccgctgatgggatgtgagctgtgacttttgggagaaggctttcccacactggctacaattataaggtttttctcctgtatgagttctgtgatgtgtaataaactgagacttctggggaaaggttttgccacaattaccacagccaaaggctatgtctcttatatgtctgctctgatgtttaatgagacttggtttcttactgaagcgcttcctacattcactgcattcatagagtttctcccctaaacgatttctatgatatatgataatctgtgactttttatagctctctttatatttatcacagtcatagtattttaaccaggtatcagtatcctcaggcttggaatggagaaaaaaattatcaaacacattaaagtcatctgattctgcttttccataatctccttttggaataagcaaatctaaatgatgttttaaaatcaatccatctaagtcaccttcactgtttgatttccttaaaggaacaaagttcatgttcagattgaaattttttccaaatgcatcacattcatgacctctttttataattttaagcttgtcttggttatcctggtgccacatcatgttaccatctactttccagacttctggagaatctgaacttggaatttctccatctcctacccacggctcttctccttgctccaatttgaagatgacatctggtttcataacttcataccccagtgacactaggctgctatagttctccaacatcacatccttgtataaattcttctgagagggatccagtagctgccactccttttgggtgaagtccacagataaatcgtcaaatgagaatgactcctgtaacatggtcattttctgctgctgtacgagatgatcagcaaggctgagatcggttctactgtgcgtctcttctgcttctgccccaaaactgtggagtgaggtctcagctaggtcttctacactgagaatgaattcctggttccaggaactcctttcttatctcacatgagcaggcttatttgtagggaccaggatctgtggacttcgggagaaatgtacttcaactggtatattcacattgcacatgaaatctctttctctcttgctaggaacttggaattcacgatcatctaaggccagaggtacgcttgctatataactgaaacagcactctcagggaaacagaatatagtaaaatggaacagtggaagcctaggtctaaaagacgccgccgccgagtcgcgcccgcgcgcccgcggcctcgcgatcacgtgacaccgcccgtcccccgtgtcccgcgcacgcgcccaaaccgtcggcctttgtgcgctcccgggcggctccgaacgggccgggacgagtcggggactgcacacgcgcacactcgcacgcgcgcacacgcgtacactcccctctcacgtggcagcgaaggacaaagaggaagaacgggccacctgcaagcatt

SEQ ID NO: 15590 - RNA, 4897 nt, Homo sapiens
  source 1..4897: mol_type = other RNA
gctgggattacaggcatgagccactgtgcccagccaggaagttcatacacttgagtatgaacaaaaagttggaaaattaaatgctttaaaattacagcatggaaagacagaattatttggctgttgaactggtattctggtttagaaaattattcatttatttaaaattccaactttcccaaaatgttgcaaaatcaataattaaaggagaaaatattgtttaaggtaaaggtgcaaaataccatactgatacaacaatttgaacataaaaggagaagtcttgagtttttctaagtttgcaatcaagctcaatattggacttttctaaatttcatcagcatacaaaaaatattaactttgccaagcaacattattgagagaacattacaaaatccttacttagctaagggatggttcatgcatttttatggaaatatataatggtaagttctcaatgtgaagttttccatggggataatgcaactagtgaaacaaagtcaaatacatttcaaatgataaaatggaaatcttgtttccttatacagatagttcctgacttaagaggatgtgacttacagtttctcaacattacaatggtatccatacactactatttttcaccttcagtattcaataattacatcagatattcaacacctttttataaaatagatgatgcattagaatgtgttctgagaatgtttaaggtaggctacgctaagctatgatgtttggtaagttgggtgtattaaatgcatttttgacttacaatgttttcaacttacaatgggtttattgggaggtaaccccactgtaagtccaggatcatctgtacttttccagggaccacagaaatttgctagaagataaaataggcatccttgaatgtcaaaaatgtttttccagcacaaaattccctaatactttacatcttcagaaatgtgattttttaataattcatttatccatctaatttttacaagatattttatgcaacacaaaaagcataacagcagcacaaaatatccatgatactttatcacagtaaattaaaatagtgacatttgggttacatatcacttaagatacatatatatatactatatggaggcacctcactaaatgagaaaaagatttaatacagcactactttatttcatttagtttgggtgttgtaatgtagttcacacacctttattttgctcattcagttatatattactatggttattctgtggttcctgcctttgcatatttattttatataaactgttactcagactctgaggatgcagaagacttacacaatgttggcttcagttactgaatagaaaggtccataaaaacaaaagaccccttatgtatgtctataagttaaaagaaacgggttatcacttaaggtacttattcatgtagtcatgttacatgagtttccattttttatattattgttaaaaaataaaaaccagtggtgtgtagtgttgtcttcacagacatcagaggcactaaaaggcatatgcatttcatactcccaattacattaaattataggtaagtccaaaacacaaaacatacgtgacactagaagataagccacaaataccactaagaaatgtcttagatgtttcaataaccaatttattcacgtatttttaaaacttcacacttcaaagtgaacatctgtcaaccacttagaattgggtatttttggtacccatgtctacaaaaagtgtatggcttcccttgacagtactatactgaggggcaagtgttcccagtgtctttaaattgttaggttctccataatatgaattctccaaaatacaaaatagtctcgttacttgttgcactgtcccatatttagtactttcatagaacttcattcctaagagcattttcttatgtacaatgaactgtcatttcttaaaaatattgcctcatttcccgcattcatggggttttccctcatccccagtgggaatatttctaatagcttaagagacttgacttctggaaggcttttggacattcacaggattcttctttgctgtgaatgttctactctataaggcttgtctatggttttaaaagtttttgagatccactgcagtcataggttcactctactctatgaattatgatcggctttccatacaccacctcatttagagttctcatcctcatggagtacaaacacctaacatgacgtgactgtctacaaacgttatcataattgcatttcctgaagtccaagatgatctgtcaaagactactattaactgtattcctaggatttttttactgtatgagttctctgatgattgatgagctgtgacttctgtgagaaagctttcccacattcaatgcatcgataaggcttctctcctgtatgaattctctgatgattaaccagctgtgacttctgagagaaggccttcctacattcactgcatccatagggtttctcacccgtatgtgtcctttgatgtggtataaggtgtgacttccgagagaaagctttgccacactcactgcattcaaaaggcttctctcctgtatgtattctctgatgattgatgagacttgacttctccctgaaggcttttctacattcattgcattcataaggtttttctcctgtatgagttctcagatgtctaattagctccgacttctcaaaaaaagctttcctacaaagactgcattcatagggtttctctccagtgtgaattctctgatgggtatttagctgtgatttctgggagaaagctttttcacagtccctgcattcatacggtttttctccagtatgagttctctgatgagttgcaagacttgacttctcaccaaaggccttcccacattcactgcattcatagggtttctcccctgtatgtgtcctctgatgtgatatgagatgtgacttctgacaaaaggctttcccacattcactgcatacatatggtttttctcctgtatgaattctttgatgattagtgagacttaatttttcactgaaagctttcccacactcactgcattcatacggtttttctcccgtatgagttctctgatgtctaacgagctgtgatttcctgctgaaggctttcccacatttactgcatataaagggtttttctcctgtgtgtgtcatctgatgtgatatgagatgtgacttctgggagaaggccttcccacactgaatgcatccatgaggtttctctcctgtatgtgttctctgatgattaatgagactcgacctctctctaaatgctttcctacactcgctgcattcatagggtttctctccagtatgaattgtctgatgtctaataagctctgacttctcaaagaatgcttttctacaatcactacatccaaagggttttgttcctgtgtgagttctgtgatgtgtaacgagttgtgacttcctgctgaaggctttcccacattccctgcattcaaaaggcttctcaccggtatgaattctctgatggttaatgagattggacttttcactaaaggccctcccacattcattgcatccatagggtttctctcctgtgtgtgttctccaatgcgatatgagatgtgacttccgggagaaggctttcccacattcaccacactcataaggtttctctcctgtatgtgtccgctgatgggatgtgagctgtgacttttgggagaaggctttcccacactggctacaattataaggtttttctcctgtatgagttctgtgatgtgtaataaactgagacttctggggaaaggttttgccacaattaccacagccaaaggctatgtctcttatatgtctgctctgatgtttaatgagacttggtttcttactgaagcgcttcctacattcactgcattcatagagtttctcccctaaacgatttctatgatatatgataatctgtgactttttatagctctctttatatttatcacagtcatagtattttaaccaggtatcagtatcctcaggcttggaatggagaaaaaaattatcaaacacattaaagtcatctgattctgcttttccataatctccttttggaataagcaaatctaaatgatgttttaaaatcaatccatctaagtcaccttcactgtttgatttccttaaaggaacaaagttcatgttcagattgaaattttttccaaatgcatcacattcatgacctctttttataattttaagcttgtcttggttatcctggtgccacatcatgttaccatctactttccagacttctggagaatctgaacttggaatttctccatctcctacccacggctcttctccttgctccaatttgaagatgacatctggtttcataacttcataccccagtgacactaggctgctatagttctccaacatcacatccttgtataaattcttctgagagggatccagtagctgccactccttttgggtgaagtccacagataaatcgtcaaatgagaatgactcctgtaacatggtcattttctgctgctgtacgagatgatcagcaaggctgagatcggttctactgtgcgtctcttctgcttctgccccaaaactgtggagtgaggtctcagctaggtcttctacactgagaatgaattcctggttccaggaactcctttcttatctcacatgagcaggcttatttgtagggaccaggatctgtggacttcgggagaaatgtacttcaactggtatattcacattgcacatgaaatctctttctctcttgctaggaacttggaattcacgatcatctaaggccagaggtacgcttgctatataactgaaacagcactctcagggaaacagaatatagtaaaatggaacagtggaagcctaggtcttgaactcacaaaagacgccgccgcc

SEQ ID NO: 15591 - RNA, 4740 nt, Homo sapiens
  source 1..4740: mol_type = other RNA
gctgggattacaggcatgagccactgtgcccagccaggaagttcatacacttgagtatgaacaaaaagttggaaaattaaatgctttaaaattacagcatggaaagacagaattatttggctgttgaactggtattctggtttagaaaattattcatttatttaaaattccaactttcccaaaatgttgcaaaatcaataattaaaggagaaaatattgtttaaggtaaaggtgcaaaataccatactgatacaacaatttgaacataaaaggagaagtcttgagtttttctaagtttgcaatcaagctcaatattggacttttctaaatttcatcagcatacaaaaaatattaactttgccaagcaacattattgagagaacattacaaaatccttacttagctaagggatggttcatgcatttttatggaaatatataatggtaagttctcaatgtgaagttttccatggggataatgcaactagtgaaacaaagtcaaatacatttcaaatgataaaatggaaatcttgtttccttatacagatagttcctgacttaagaggatgtgacttacagtttctcaacattacaatggtatccatacactactatttttcaccttcagtattcaataattacatcagatattcaacacctttttataaaatagatgatgcattagaatgtgttctgagaatgtttaaggtaggctacgctaagctatgatgtttggtaagttgggtgtattaaatgcatttttgacttacaatgttttcaacttacaatgggtttattgggaggtaaccccactgtaagtccaggatcatctgtacttttccagggaccacagaaatttgctagaagataaaataggcatccttgaatgtcaaaaatgtttttccagcacaaaattccctaatactttacatcttcagaaatgtgattttttaataattcatttatccatctaatttttacaagatattttatgcaacacaaaaagcataacagcagcacaaaatatccatgatactttatcacagtaaattaaaatagtgacatttgggttacatatcacttaagatacatatatatatactatatggaggcacctcactaaatgagaaaaagatttaatacagcactactttatttcatttagtttgggtgttgtaatgtagttcacacacctttattttgctcattcagttatatattactatggttattctgtggttcctgcctttgcatatttattttatataaactgttactcagactctgaggatgcagaagacttacacaatgttggcttcagttactgaatagaaaggtccataaaaacaaaagaccccttatgtatgtctataagttaaaagaaacgggttatcacttaaggtacttattcatgtagtcatgttacatgagtttccattttttatattattgttaaaaaataaaaaccagtggtgtgtagtgttgtcttcacagacatcagaggcactaaaaggcatatgcatttcatactcccaattacattaaattataggtaagtccaaaacacaaaacatacgtgacactagaagataagccacaaataccactaagaaatgtcttagatgtttcaataaccaatttattcacgtatttttaaaacttcacacttcaaagtgaacatctgtcaaccacttagaattgggtatttttggtacccatgtctacaaaaagtgtatggcttcccttgacagtactatactgaggggcaagtgttcccagtgtctttaaattgttaggttctccataatatgaattctccaaaatacaaaatagtctcgttacttgttgcactgtcccatatttagtactttcatagaacttcattcctaagagcattttcttatgtacaatgaactgtcatttcttaaaaatattgcctcatttcccgcattcatggggttttccctcatccccagtgggaatatttctaatagcttaagagacttgacttctggaaggcttttggacattcacaggattcttctttgctgtgaatgttctactctataaggcttgtctatggttttaaaagtttttgagatccactgcagtcataggttcactctactctatgaattatgatcggctttccatacaccacctcatttagagttctcatcctcatggagtacaaacacctaacatgacgtgactgtctacaaacgttatcataattgcatttcctgaagtccaagatgatctgtcaaagactactattaactgtattcctaggatttttttactgtatgagttctctgatgattgatgagctgtgacttctgtgagaaagctttcccacattcaatgcatcgataaggcttctctcctgtatgaattctctgatgattaaccagctgtgacttctgagagaaggccttcctacattcactgcatccatagggtttctcacccgtatgtgtcctttgatgtggtataaggtgtgacttccgagagaaagctttgccacactcactgcattcaaaaggcttctctcctgtatgtattctctgatgattgatgagacttgacttctccctgaaggcttttctacattcattgcattcataaggtttttctcctgtatgagttctcagatgtctaattagctccgacttctcaaaaaaagctttcctacaaagactgcattcatagggtttctctccagtgtgaattctctgatgggtatttagctgtgatttctgggagaaagctttttcacagtccctgcattcatacggtttttctccagtatgagttctctgatgagttgcaagacttgacttctcaccaaaggccttcccacattcactgcattcatagggtttctcccctgtatgtgtcctctgatgtgatatgagatgtgacttctgacaaaaggctttcccacattcactgcatacatatggtttttctcctgtatgaattctttgatgattagtgagacttaatttttcactgaaagctttcccacactcactgcattcatacggtttttctcccgtatgagttctctgatgtctaacgagctgtgatttcctgctgaaggctttcccacatttactgcatataaagggtttttctcctgtgtgtgtcatctgatgtgatatgagatgtgacttctgggagaaggccttcccacactgaatgcatccatgaggtttctctcctgtatgtgttctctgatgattaatgagactcgacctctctctaaatgctttcctacactcgctgcattcatagggtttctctccagtatgaattgtctgatgtctaataagctctgacttctcaaagaatgcttttctacaatcactacatccaaagggttttgttcctgtgtgagttctgtgatgtgtaacgagttgtgacttcctgctgaaggctttcccacattccctgcattcaaaaggcttctcaccggtatgaattctctgatggttaatgagattggacttttcactaaaggccctcccacattcattgcatccatagggtttctctcctgtgtgtgttctccaatgcgatatgagatgtgacttccgggagaaggctttcccacattcaccacactcataaggtttctctcctgtatgtgtccgctgatgggatgtgagctgtgacttttgggagaaggctttcccacactggctacaattataaggtttttctcctgtatgagttctgtgatgtgtaataaactgagacttctggggaaaggttttgccacaattaccacagccaaaggctatgtctcttatatgtctgctctgatgtttaatgagacttggtttcttactgaagcgcttcctacattcactgcattcatagagtttctcccctaaacgatttctatgatatatgataatctgtgactttttatagctctctttatatttatcacagtcatagtattttaaccaggtatcagtatcctcaggcttggaatggagaaaaaaattatcaaacacattaaagtcatctgattctgcttttccataatctccttttggaataagcaaatctaaatgatgttttaaaatcaatccatctaagtcaccttcactgtttgatttccttaaaggaacaaagttcatgttcagattgaaattttttccaaatgcatcacattcatgacctctttttataattttaagcttgtcttggttatcctggtgccacatcatgttaccatctactttccagacttctggagaatctgaacttggaatttctccatctcctacccacggctcttctccttgctccaatttgaagatgacatctggtttcataacttcataccccagtgacactaggctgctatagttctccaacatcacatccttgtataaattcttctgagagggatccagtagctgccactccttttgggtgaagtccacagataaatcgtcaaatgagaatgactcctgtaacatggtcattttctgctgctgtacgagatgatcagcaaggctgagatcggttctactgtgcgtctcttctgcttctgccccaaaactgtggagtgaggtctcagctaggtcttctacactgagaatgaattcctggttccaggaactcctttcttatctcacatgagcaggcttatttgtagggaccaggatctgtggatgaactcacaaaagacgccgccgccgagtcgcgcccgcgcgcccgc

SEQ ID NO: 15592 - RNA, 1913 nt, Homo sapiens
  source 1..1913: mol_type = other RNA
gctgggattacaggcatgagccactgtgcccagcccactcctgagcttgttacgtgtcctctgggggagcccccagcatcactgctggccccagctcccagccagggccctaggtacacaggcaggagggactggtgccatcattctacccttgcagggtgccaaggctgtgagtgagctcaccagaggaggaggggaatcagtgggtggccccacagccagggcctgagctcaggaaaagcggcactgtggcgggtgtgtggtatgtcaggagcccagaagctgctgtcctaggcccctttcctcctgcacagcatgatgtggtgtaaatgaggggtctcagctgagggacattttgctgagtgtcagaagcaaagggagggttaggaaaccctggggaaaagggaatgtcaaggtagggaggcaaggcctttctacatgaggaccacgggcagggcagcagagtcccagagaggtccagtgggcaccagggagggctgccatcttcctcagtggggcagaccctgcctgatggcacagtggtagacagcacctccccaccccactccctaaccgacacaaatctccacatacaaccaggtcctgtcctcacctcaccatgacaaccagcacccagctcaggcctgcatggccctggtgtggacccaaaggtggggtgtggggtgaggatgaggaaggcagcgtccatgtcctttgagggcaaggctggcccccaagtggagctccggcccagaggagacataggctccagaccagagaggccaggagctggtagagtgaggcctccctctgccaccccttcccctcccccgcccatccaggggagacttgggaagcaggggaggagcgcccatcactttccaccccgggagagtgccgagggggctccaggctgggtggccatgatgtggtagatggattcccggaagcgctggtccctgctgagccgcttggccacctcctttagctcctccatgttgttggcatccagctgggaggtcatgaaggactgggacggcttcatgtcattccaggaggtgctggaccggcgtcggtggaagcggcagctcttgatgcggcgagtggctgccttatggatgtacacggagttcttcatgatcacaggcatcttggcctccagctcggcattccggatgcactcctcaaagaaccttttcagatggctcacatcagcccgcatcctctcctccttctccttattccgcaccttggaattcagcccctgttccaggcttcgcaaggccccttctgcctcccggagacgcctctccaggtccatgcggaccttcacctcagccttgagctcccgctcagcctgctgcttctctgccgtcagctcctgcagcgagttctgcagtgcctgggactggctggagtagaactcacgctcctcctccagggcccgtgagcgctcctcgttctccttcatccgcttctctgccaggagcttctcctctaagagctgctgcatcttctcctcgatctgccggaggttgctatggaggcccccactgggagggggctgctcactctgattggccagtgtctgcaggtggttctcgttctcctccagcatttccagggttttcttcttctctatggagagttcctccagtgtctgctgcaaggactccgtgaggtgcctcagttcctttttctcttgttctacacccttaaggcatcttgcagtcagttccagctccctcttgatctgctcctgctccattctcagctcctgcaccacctcctcgaactgctgcttctcggcctccagcacctggttaaggcgctcaagctcaaacatttcccgttacttgatattacgctgggatatccttttgtagttgaaaacgggggagggtcaatgatta

SEQ ID NO: 15593 - RNA, 2969 nt, Homo sapiens
  source 1..2969: mol_type = other RNA
gctgggattacaggcatgagccactgtgcccagcccactcctgagcttgttacgtgtcctctgggggagcccccagcatcactgctggccccagctcccagccagggccctaggtacacaggcaggagggactggtgccatcattctacccttgcagggtgccaaggctgtgagtgagctcaccagaggaggaggggaatcagtgggtggccccacagccagggcctgagctcaggaaaagcggcactgtggcgggtgtgtggtatgtcaggagcccagaagctgctgtcctaggcccctttcctcctgcacagcatgatgtggtgtaaatgaggggtctcagctgagggacattttgctgagtgtcagaagcaaagggagggttaggaaaccctggggaaaagggaatgtcaaggtagggaggcaaggcctttctacatgaggaccacgggcagggcagcagagtcccagagaggtccagtgggcaccagggagggctgccatcttcctcagtggggcagaccctgcctgatggcacagtggtagacagcacctccccaccccactccctaaccgacacaaatctccacatacaaccaggtcctgtcctcacctcaccatgacaaccagcacccagctcaggcctgcatggccctggtgtggacccaaaggtggggtgtggggtgaggatgaggaaggcagcgtccatgtcctttgagggcaaggctggcccccaagtggagctccggcccagaggagacataggctccagaccagagaggccaggagctggtagagtgaggcctccctctgccaccccttcccctcccccgcccatccaggggagacttgggaagcaggggaggagcgcccatcactttccaccccgggagagtgccgagggggctccaggctgggtggccatgatgtggtagatggattcccggaagcgctggtccctgctgagccgcttggccacctcctttagctcctccatgttgttggcatccagctgggaggtcatgaaggactgggacggcttcatgtcattccaggaggtgctggaccggcgtcggtggaagcggcagctcttgatgcggcgagtggctgccttatggatgtacacggagttcttcatgatcacaggcatcttggcctccagctcggcattccggatgcactcctcaaagaaccttttcagatggctcacatcagcccgcatcctctcctccttctccttattccgcaccttggaattcagcccctgttccaggcttcgcaaggccccttctgcctcccggagacgcctctccaggtccatgcggaccttcacctcagccttgagctcccgctcagcctgctgcttctctgccgtcagctcctgcagcgagttctgcagtgcctgggactggctggagtagaactcacgctcctcctccagggcccgtgagcgctcctcgttctccttcatccgcttctctgccaggagcttctcctctaagagctgctgcatcttctcctcgatctgccggaggttgctatggaggcccccactgggagggggctgctcactctgattggccagtgtctgcaggtggttctcgttctcctccagcatttccagggttttcttcttctctatggagagttcctccagtgtctgctgcaaggactccgtgaggtgcctcagttcctttttctcttgttctacacccttaaggcatcttgcagtcagttccagctccctcttgatctgctcctgctccattctcagctcctgcaccacctcctcgaactgctgcttctcggcctccagcacctggttaaggcgctcaagctcctctctctgctccctctgaaggcagagttcttcggtctcttccatcagtttgtctaaatactcctgcttttccttagccaactgcagcccctgggcctccaggcttttgatcatggcttctcccagctgggcattcttccaggtcaccttcccagactcctgcagcatctccagccactgggtctgctcaaactccgactcagcagcaagcaagatgttcccatggaagtcctggtgggagatcttcatggcatagggcatgctaggctcttccttgggctccaccaggcagccccccagagggatgacgcccttaggatgtatattgaagtatttattggtttcaaagctctttttttcgctctcagagtagtaaagcagaaagctctctttgatgatgaaaaacaattccacaatccagagataattacagttgaaatttgagggtataattttctgaactagttgtattcatttatctctgcccttctttttcactatccttatattacaattttcgaaaggagtatctgccacatgcagtctggtaaactgcttttcatacctgaaattaatcatgaacatatttgtaattacatttttgatctcatagtattccattgtattgcttttccataatttaactaatctgttattgtttaactcacggctctgaacactggataaaaacatggtcctatccatgaactatctcccttgtcttaactaactccacaagtcctcccaaaacatgtgaatgcctgacctcttcatgaataactgtgtttatttcttggcctactgacattcaagaatgtggcctttatttctcgaaggagtggggttgatcgaaaccagcacagaaggctgtgtatcaagatgaggtattggagaactacaggaatttggctcactggatagacatcgttccaccatggttgaagatgtaactcctgttcagaaatgatttattagtggtgaaattccaaggagcttctgaggtgcctcctgttcacaaatagttgagatttgagggttgataataagcagctctactgaccctcacctgaaactccatctcccccaaatccccacctttttttttgagacagagtctggctctatcacc

SEQ ID NO: 15594 - RNA, 2633 nt, Homo sapiens
  source 1..2633: mol_type = other RNA
gctgggattacaggcatgagccactgtgcccagcccactcctgagcttgttacgtgtcctctgggggagcccccagcatcactgctggccccagctcccagccagggccctaggtacacaggcaggagggactggtgccatcattctacccttgcagggtgccaaggctgtgagtgagctcaccagaggaggaggggaatcagtgggtggccccacagccagggcctgagctcaggaaaagcggcactgtggcgggtgtgtggtatgtcaggagcccagaagctgctgtcctaggcccctttcctcctgcacagcatgatgtggtgtaaatgaggggtctcagctgagggacattttgctgagtgtcagaagcaaagggagggttaggaaaccctggggaaaagggaatgtcaaggtagggaggcaaggcctttctacatgaggaccacgggcagggcagcagagtcccagagaggtccagtgggcaccagggagggctgccatcttcctcagtggggcagaccctgcctgatggcacagtggtagacagcacctccccaccccactccctaaccgacacaaatctccacatacaaccaggtcctgtcctcacctcaccatgacaaccagcacccagctcaggcctgcatggccctggtgtggacccaaaggtggggtgtggggtgaggatgaggaaggcagcgtccatgtcctttgagggcaaggctggcccccaagtggagctccggcccagaggagacataggctccagaccagagaggccaggagctggtagagtgaggcctccctctgccaccccttcccctcccccgcccatccaggggagacttgggaagcaggggaggagcgcccatcactttccaccccgggagagtgccgagggggctccaggctgggtggccatgatgtggtagatggattcccggaagcgctggtccctgctgagccgcttggccacctcctttagctcctccatgttgttggcatccagctgggaggtcatgaaggactgggacggcttcatgtcattccaggaggtgctggaccggcgtcggtggaagcggcagctcttgatgcggcgagtggctgccttatggatgtacacggagttcttcatgatcacaggcatcttggcctccagctcggcattccggatgcactcctcaaagaaccttttcagatggctcacatcagcccgcatcctctcctccttctccttattccgcaccttggaattcagcccctgttccaggcttcgcaaggccccttctgcctcccggagacgcctctccaggtccatgcggaccttcacctcagccttgagctcccgctcagcctgctgcttctctgccgtcagctcctgcagcgagttctgcagtgcctgggactggctggagtagaactcacgctcctcctccagggcccgtgagcgctcctcgttctccttcatccgcttctctgccaggagcttctcctctaagagctgctgcatcttctcctcgatctgccggaggttgctatggaggcccccactgggagggggctgctcactctgattggccagtgtctgcaggtggttctcgttctcctccagcatttccagggttttcttcttctctatggagagttcctccagtgtctgctgcaaggactccgtgaggtgcctcagttcctttttctcttgttctacacccttaaggcatcttgcagtcagttccagctccctcttgatctgctcctgctccattctcagctcctgcaccacctcctcgaactgctgcttctcggcctccagcacctggttaaggcgctcaagctcctctctctgctccctctgaaggcagagttcttcggtctcttccatcagtttgtctaaatactcctgcttttccttagccaactgcagcccctgggcctccaggcttttgatcatggcttctcccagctgggcattcttccaggtcaccttcccagactcctgcagcatctccagccactgggtctgctcaaactccgactcagcagcaagcaagatgttcccatggaagtcctggtgggagatcttcatggcatagggcatgctaggctcttccttgggctccaccaggcagccccccagagggatgacgcccttaggatgtatattgaagtatttattggtttcaaagctctttttttcgctctcagagtagtaaagcagaaagctctctttgatgatgaaaaaccgccgggaccacttggccgacggcctgccgaaaggcctcttccacagcacgccgtagagctgcactttggtgctgatatccagggcgtccgagtcagcctgctccagggacggcgagggcgacaccgagttggacttggacgtgaacatcctgcctcagcggggctgtgcccggcccggaccccacctccccggggtcagcagggactcggggcgagaggcgagggcggagccgtcggagagcgtcccagcgagcagagaagcagagcggcccggcccggagctgcagcatcaaagcgcgctgggcactggacgcggcaccaagggggcgcagggcgcgtagccggcggcttgggctccggattgcagagggccgggcgggaactcc

SEQ ID NO: 15595 - RNA, 2053 nt, Homo sapiens
  source 1..2053: mol_type = other RNA
gctgggattacaggcatgagccactgtgcccagcccactcctgagcttgttacgtgtcctctgggggagcccccagcatcactgctggccccagctcccagccagggccctaggtacacaggcaggagggactggtgccatcattctacccttgcagggtgccaaggctgtgagtgagctcaccagaggaggaggggaatcagtgggtggccccacagccagggcctgagctcaggaaaagcggcactgtggcgggtgtgtggtatgtcaggagcccagaagctgctgtcctaggcccctttcctcctgcacagcatgatgtggtgtaaatgaggggtctcagctgagggacattttgctgagtgtcagaagcaaagggagggttaggaaaccctggggaaaagggaatgtcaaggtagggaggcaaggcctttctacatgaggaccacgggcagggcagcagagtcccagagaggtccagtgggcaccagggagggctgccatcttcctcagtggggcagaccctgcctgatggcacagtggtagacagcacctccccaccccactccctaaccgacacaaatctccacatacaaccaggtcctgtcctcacctcaccatgacaaccagcacccagctcaggcctgcatggccctggtgtggacccaaaggtggggtgtggggtgaggatgaggaaggcagcgtccatgtcctttgagggcaaggctggcccccaagtggagctccggcccagaggagacataggctccagaccagagaggccaggagctggtagagtgaggcctccctctgccaccccttcccctcccccgcccatccaggggagacttgggaagcaggggaggagcgcccatcactttccaccccgggagagtgccgagggggctccaggctgggtggccatgatgtggtagatggattcccggaagcgctggtccctgctgagccgcttggccacctcctttagctcctccatgttgttggcatccagctgggaggtcatgaaggactgggacggcttcatgtcattccaggaggtgctggaccggcgtcggtggaagcggcagctcttgatgcggcgagtggctgccttatggatgtacacggagttcttcatgatcacaggcatcttggcctccagctcggcattccggatgcactcctcaaagaaccttttcagatggctcacatcagcccgcatcctctcctccttctccttattccgcaccttggaattcagcccctgttccaggcttcgcaaggccccttctgcctcccggagacgcctctccaggtccatgcggaccttcacctcagccttgagctcccgctcagcctgctgcttctctgccgtcagctcctgcagcgagttctgcagtgcctgggactggctggagtagaactcacgctcctcctccagggcccgtgagcgctcctcgttctccttcatccgcttctctgccaggagcttctcctctaagagctgctgcatcttctcctcgatctgccggaggttgctatggaggcccccactgggagggggctgctcactctgattggccagtgtctgcaggtggttctcgttctcctccagcatttccagggttttcttcttctctatggagagttcctccagtgtctgctgcaaggactccgtgaggtgcctcagttcctttttctcttgttctacacccttaaggcatcttgcagtcagttccagctccctcttgatctgctcctgctccattctcagctcctgcaccacctcctcgaactgctgcttctcggcctccagcacctggttaaggcgctcaagctcctctctctgctccctctgaaggcagagttcttcggtctcttccatcagtttgtctaaatactcctgcttttccttagccaactgcagcccctgggcctccaggcttttgatcatggcttctcccagctgggcattcttccaggtccctttctcctccagaatctcaacttgcattcactctggcacccatggctctgggcatgtcaccagcac

SEQ ID NO: 15596 - RNA, 6590 nt, Homo sapiens
  source 1..6590: mol_type = other RNA
gctgggattacaggcatgagccactgtgcccagccctattttgtagttttaaatagctcatgttgctacctgagccccagttttctcatcagaatattagggctcacaacatttattatgtttttgtgatgagtcaaataaaacaaaatgtgtaacagttctttgagaaagcaatgcattttatcaatacatggcataaccttaataatagcctcacaagatattatacttataatatttgtaaataatactatcacaaaaatcttagtcctatgatataattgtcctggagataatataaaataatgcaagtttatgacccaactaaaatacatgttattgaaactcaagaatagacctagtattgtagatgttagtcttagaggttgagattgtgtattttagaaacttcaaagattatagaaaaattttaagaaaaaatgtgtaaaaatggggaaatctttttatttacgagttacctggaaatgtttaatactcaatgtgataaataatgttgtcctttctaattgaaactacttttttgtacacatattggcacagcaaattgctatggctggaggttggacactttcaacagttagttatttcatgcatacatataatttgtaaagccgacaaaaaagaaaagataaaaactctaagtagaaaatagaattttataactacgttttacagattattccaagagatatcattggttattttattcttttgaaaatattacttatttaaacaactaaaaaaaccggtaaagcctgatataatttcaacattagaaagaataaattattgaaaaatatgtagaacaaaaacaccatcttaatgccattggtaccactatactgttgagcaagtattatatgaggtattgaacattgcacataattatacacttaggatttgagattgtagataaaccagttgttcaaggccactaaaatactgaaaaaggattatgattattaacagtgaggaggaaaatacaactataaaagcccttcaaactcaaatctggaaatggtaattttactcaaaaatataccacaactactaagagattttagtaattcatgacacaaaacaagacatccacctctaatttttttcttatctattacatgaattcagtggtgatagaccacatatttgggacctccatcgcagtgtgatatttagtattgttatattttagaagttactcatttaattaaggattttataaacgtgatatgtggtaactggattttatcatttctgataaatggaaaaagtttagattttatactaaaagtattatcatgcctattcacatcatgtaaaatatttaaaattcatgtattttaattgaatgaagtgctgaaaaatttaggtatgactaataggtattacttgcttatatgataaaattcagttttaggtggtactttattctatagattcggaaatagctcctcttttctactaatttaaaataattctatggctctggttcttaaaatgtctaattattttcactattcagtgcgtactgttagaatatatttctttcaatgatttgtaagatttggtggagtgaaaaacctcaggaaaataagacgtgatttacaaacatttggctatgtagagtagttgcattggtattttatactggtaaacttaaaatatgctaattttgaagcatctaagcaacgtttggagagctggcctactgggtgagaataccatttaaaaacatttgtgttacacaacacacagccatgaaaatggctattcaaaattcccaggtagaacacagttgtcagtgccaaaagaaaagctttgtacattaacacaagaaaaggaacttttcatcttaagggatggcacaactggcacaaaaggtcattaaatgctaatagacccacttgaggtatgctcgcttaatggaggattagagcaaaacagacttaaaagaccaacatgcagagaatttttttaactctctggactactcagcataaggtaggaaaacaaacaagatggaaaataaactctttttcagcactaataattataagtttgcataattgtttcatgcaaaaggaactttgacagaaaacgatggcaaaatctataggcaagactgacacaggagaactggaatagtagtttatacaaaaattttgtttgtattcatcttcatgtagcagaatagaccactgttcaagaagtagatgaaaaattcataacagttgagaaatttagttaggacatagaaagaataatgttgagataaattccttgaagccttttgcaactgtccttaagtttataaaaagagataaattttctttgatctgaagacattctttgtacatgtgcagtgtacaacatactatatacatatggggcttccctatgtacatatacatatgcatacactatctatatgccttttaaaatgtatacacagctttaactcaaagaaaatgagttagcaacacagtaatcattgccagacaatccaagtgctgaaataagtgatgttcatcatgtcaagggctattttacctctcacattgcccaaaattgagaatatcatttctgtttttagtttttctttcattgcaatactgattgtcatatataatctttgtgcttttgcataatgcccatcctaggtgtaacacatattcacacacaacactggacgtttgaaataagcatgctggaacacaggcaggacaatatatccatgcacagatattctgaatatgtttttccaaattgactgtaacatcaacatgcatcactatcatatttggtcctgtacagcaaggaatgtacagctgaagcaatcatggctagtttcacttgcaagagtttctttagagaggaacacccagtagagaaacagaacagaatgaatgaaacaaataaaaaatatcccccaaaaccaaaaaataaaaactaaaaaaaaaattcctcccacacgttaacactgaaaatctggccattttctaggtagtacattttcctcattccacaaaaagcgtgtcttctcataaacttctgagttgaattgtttgtttataagatacatatattagtgtcttagagcttttcctaaccattggaaaagctcgtcttggtaaagcattttccagcgcacattggcttcgacagtttccacagctcgtgagaaagaagcagcagctaccccatcatagtttttcatgaagttcttgagctctttgagttcaccttcagtattaagaaattctgtgacaccactgatgagtttggaattcataaacaatgcttctccatacctggtatttaatatcttccatttatccctgaaaaacttccaggcaaggtctcgaccatgtggatttcgagctacatggattatgacatcaattgcatcttgatccagcaccacctcagaattcagtgacagatttagaagcctgtttaataaattcctgtcatcactgcaagttaaggcttccaataatattttcttctcagaaactgctgtggtggaatggaatttcatccatatgaattcccagacatcctcatccagtagtgacactcctgtacagtatacgatgtctctaacatttagtggtattctgttcctgttgctggaaatccaatctgaaataagtgttgatgcctgttggtgacagtgcttgttgccaaaactgcaggccagcattataacttctctacgtagttcttcatgttggtaggatgcttgaacaagagatccattaaaattatttttcggccacccaagcttgatatatgttgttgcaacttgctttaaaatatattcattgaaaatgttgtagttttccatgcggtccagtaatttatctagaggataaagagctcggctggcagcatgccaaggaagaaaatccttctcctcagacaggtatctgataatctccagaggaatattctgaggcaaatagccagccctggctaggctgaaggcatcatcgatcaagcccgctcggttactgacagaaagaacctcatgattccggattaattgatcaattaataatctccagttccttaggtcatagttgactctaaaatagccagtttgattgatgttccccagcagccagcttcctttgtccaaataagttattctgtggtgctctgatttgttagacacccaaataattgcttctgaagacacatggcttctatttcctaccacaatagttaatggaatctgccacaggtaactgttattctgaagtttaagtgctttagttttagcactgatatcatagataaaatgctgttgggtaattattattctattttctgctgttgtgtttcccaagatggtgataacaggataacccatctggagtgtccactgatccattacttcttgtatatttacatatttcccatttctttttaaagcctccgataatgtattccagagatcatttctggctgcattaccatacttatgaatggttaaataatcttgcaaacccctctggaaaactgaatggcccataaaattagccagcattcttattaaagcagcaccctttttatatgcgatccagtcaaacaccctgtcaatatctgttgcctgcagcacttcctgtgatactggatgggaactggccaaaccgtccagcagcatcacttcatgcagaacatcggtcagaaacctctgcttttccatgttccagccaggatagaggtagtctgtaccaacaaattcaaagtagtgagcaaacccttccttcagccacacgtcttcccaccacacaggcgtcacaaggtcaccaaaccactggtgacatatctcatgaacaatgaccatggtgacatccagcaaataagaaatagatgaaacactgggatccagcagtattctttgttccacaaaaatacttagtccccagttctccatagcagcatacggatgcttaggcacagctaaaagatctagttttggcaaggaatagggcactttaaagtagtcttcataaaattctattaatctctttgttatatggagagcatagtccccggatcctcttctgatagcatcaggtcttgcatataatcgtactacaaccccactcttggtggtagtttctctgtatgtgaagttgcaaattgcccaggctaaataatatgtggacatgagaggggtctgtgaaaagtgatccgtaacccatccatcttcctcaaacacggaagtttccactggcatattagataaagataaataggttgcttgatgcttgatgctgattttgaaagtagccttgtagattggctcatcaaaacaaggaaatgcctttctggcatgtgtaggcgaaaactgagtaacaccaaggaatcttctctccccgtggagcacataggagctgcggaagaagcccaggagctcattctcgatgagcgcgttgtagataatcttcagattgtaattcctctgcgcgtccagtgtcctattcagcaccaccactaagacctgggtttgcgggtagaggaaaaaaccggctacagggacagccccgaacgcccggtcctcggccagctgcactttctccaccgccactcgggaagcgtgcagcactacgtagcgggtggcgttccggcacgcgatctccacgttgacctccccggagaaggtgaagttctccatgaaggcggtgagcatcagattgtagtgcagcggcttcaggtggcccgacaggcgcagctgcgtccacggctcccacggctcccgctcctcctccgacggcggctgggccgacgtggtccccggactggccaccccacccgcctcgggctgccaggagtccccgcctgcgtggtggttgcgccgggccgatccagggaggctcccgttgccgccgcgctccggaaagcctgaggggccaccgtcggcgcctggcgtggcactcgccccgcactcgtcgaagcgcaggctgagcagcacagcgagcattgtgaccgcgagcaatgccacgagggacacagcgaaggccagcacaagccgcttgtgtacggcgatgtggcgctccgtggtgcggggtcgcactcccactgagtctgcccacgggtcggagagccccctgctgccagcccgaagcgcggcgtcgtcttcccccatcgcggctgcgaagggtgagctgctcttctcggccccctcctcctcctcctcctcctccttcttcttcttcctcttctttttcttcttctttttcttctcctcctcttgctcccccagctcgccgtccagggccatcacaccgcctcctcctcctcccccgccccctctggcaccccccgcgggcgggccacccgggccacagccagagcaggcatcggagagctcacgcgggccgagggcgcgcgactggggatgctggcccgggttcttttaagacgggttctggacacaagcgacggcagcttccgcgacccccatcagccccgcctcactctggacaccgggctgtgagctctgggacgcgcccaacttggaaagcgtcttgcttgcccagcgcgcgctacttctc

SEQ ID NO: 15597 - RNA, 5659 nt, Homo sapiens
  source 1..5659: mol_type = other RNA
gctgggattacaggcatgagccactgtgcccagccctattttgtagttttaaatagctcatgttgctacctgagccccagttttctcatcagaatattagggctcacaacatttattatgtttttgtgatgagtcaaataaaacaaaatgtgtaacagttctttgagaaagcaatgcattttatcaatacatggcataaccttaataatagcctcacaagatattatacttataatatttgtaaataatactatcacaaaaatcttagtcctatgatataattgtcctggagataatataaaataatgcaagtttatgacccaactaaaatacatgttattgaaactcaagaatagacctagtattgtagatgttagtcttagaggttgagattgtgtattttagaaacttcaaagattatagaaaaattttaagaaaaaatgtgtaaaaatggggaaatctttttatttacgagttacctggaaatgtttaatactcaatgtgataaataatgttgtcctttctaattgaaactacttttttgtacacatattggcacagcaaattgctatggctggaggttggacactttcaacagttagttatttcatgcatacatataatttgtaaagccgacaaaaaagaaaagataaaaactctaagtagaaaatagaattttataactacgttttacagattattccaagagatatcattggttattttattcttttgaaaatattacttatttaaacaactaaaaaaaccggtaaagcctgatataatttcaacattagaaagaataaattattgaaaaatatgtagaacaaaaacaccatcttaatgccattggtaccactatactgttgagcaagtattatatgaggtattgaacattgcacataattatacacttaggatttgagattgtagataaaccagttgttcaaggccactaaaatactgaaaaaggattatgattattaacagtgaggaggaaaatacaactataaaagcccttcaaactcaaatctggaaatggtaattttactcaaaaatataccacaactactaagagattttagtaattcatgacacaaaacaagacatccacctctaatttttttcttatctattacatgaattcagtggtgatagaccacatatttgggacctccatcgcagtgtgatatttagtattgttatattttagaagttactcatttaattaaggattttataaacgtgatatgtggtaactggattttatcatttctgataaatggaaaaagtttagattttatactaaaagtattatcatgcctattcacatcatgtaaaatatttaaaattcatgtattttaattgaatgaagtgctgaaaaatttaggtatgactaataggtattacttgcttatatgataaaattcagttttaggtggtactttattctatagattcggaaatagctcctcttttctactaatttaaaataattctatggctctggttcttaaaatgtctaattattttcactattcagtgcgtactgttagaatatatttctttcaatgatttgtaagatttggtggagtgaaaaacctcaggaaaataagacgtgatttacaaacatttggctatgtagagtagttgcattggtattttatactggtaaacttaaaatatgctaattttgaagcatctaagcaacgtttggagagctggcctactgggtgagaataccatttaaaaacatttgtgttacacaacacacagccatgaaaatggctattcaaaattcccaggtagaacacagttgtcagtgccaaaagaaaagctttgtacattaacacaagaaaaggaacttttcatcttaagggatggcacaactggcacaaaaggtcattaaatgctaatagacccacttgaggtatgctcgcttaatggaggattagagcaaaacagacttaaaagaccaacatgcagagaatttttttaactctctggactactcagcataaggtaggaaaacaaacaagatggaaaataaactctttttcagcactaataattataagtttgcataattgtttcatgcaaaaggaactttgacagaaaacgatggcaaaatctataggcaagactgacacaggagaactggaatagtagtttatacaaaaattttgtttgtattcatcttcatgtagcagaatagaccactgttcaagaagtagatgaaaaattcataacagttgagaaatttagttaggacatagaaagaataatgttgagataaattccttgaagccttttgcaactgtccttaagtttataaaaagagataaattttctttgatctgaagacattctttgtacatgtgcagtgtacaacatactatatacatatggggcttccctatgtacatatacatatgcatacactatctatatgccttttaaaatgtatacacagctttaactcaaagaaaatgagttagcaacacagtaatcattgccagacaatccaagtgctgaaataagtgatgttcatcatgtcaagggctattttacctctcacattgcccaaaattgagaatatcatttctgtttttagtttttctttcattgcaatactgattgtcatatataatctttgtgcttttgcataatgcccatcctaggtgtaacacatattcacacacaacactggacgtttgaaataagcatgctggaacacaggcaggacaatatatccatgcacagatattctgaatatgtttttccaaattgactgtaacatcaacatgcatcactatcatatttggtcctgtacagcaaggaatgtacagctgaagcaatcatggctagtttcacttgcaagagtttctttagagaggaacacccagtagagaaacagaacagaatgaatgaaacaaataaaaaatatcccccaaaaccaaaaaataaaaactaaaaaaaaaattcctcccacacgttaacactgaaaatctggccattttctaggtagtacattttcctcattccacaaaaagcgtgtcttctcataaacttctgagttgaattgtttgtttataagatacatatattagtgtcttagagcttttcctaaccattggaaaagctcgtcttggtaaagcattttccagcgcacattggcttcgacagtttccacagctcgtgagaaagaagcagcagctaccccatcatagtttttcatgaagttcttgagctctttgagttcaccttcagtattaagaaattctgtgacaccactgatgagtttggaattcataaacaatgcttctccatacctggtatttaatatcttccatttatccctgaaaaacttccaggcaaggtctcgaccatgtggatttcgagctacatggattatgacatcaattgcatcttgatccagcaccacctcagaattcagtgacagatttagaagcctgtttaataaattcctgtcatcactgcaagttaaggcttccaataatattttcttctcagaaactgctgtggtggaatggaatttcatccatatgaattcccagacatcctcatccagtagtgacactcctgtacagtatacgatgtctctaacatttagtggtattctgttcctgttgctggaaatccaatctgaaataagtgttgatgcctgttggtgacagtgcttgttgccaaaactgcaggccagcattataacttctctacgtagttcttcatgttggtaggatgcttgaacaagagatccattaaaattatttttcggccacccaagcttgatatatgttgttgcaacttgctttaaaatatattcattgaaaatgttgtagttttccatgcggtccagtaatttatctagaggataaagagctcggctggcagcatgccaaggaagaaaatccttctcctcagacaggtatctgataatctccagaggaatattctgaggcaaatagccagccctggctaggctgaaggcatcatcgatcaagcccgctcggttactgacagaaagaacctcatgattccggattaattgatcaattaataatctccagttccttaggtcatagttgactctaaaatagccagtttgattgatgttccccagcagccagcttcctttgtccaaataagttattctgtggtgctctgatttgttagacacccaaataattgcttctgaagacacatggcttctatttcctaccacaatagttaatggaatctgccacaggtaactgttattctgaagtttaagtgctttagttttagcactgatatcatagataaaatgctgttgggtaattattattctattttctgctgttgtgtttcccaagatggtgataacaggataacccatctggagtgtccactgatccattacttcttgtatatttacatatttcccatttctttttaaagcctccgataatgtattccagagatcatttctggctgcattaccatacttatgaatggttaaataatcttgcaaacccctctggaaaactgaatggcccataaaattagccagcattcttattaaagcagcaccctttttatatgcgatccagtcaaacaccctgtcaatatctgttgcctgcagcacttcctgtgatactggatgggaactggccaaaccgtccagcagcatcacttcatgcagaacatcggtcagaaacctctgcttttccatgttccagccaggatagaggtagtctgtaccaacaaattcaaagtagtgagcaaacccttccttcagccacacgtcttcccaccacacaggcgtcacaaggtcaccaaaccactggtgacatatctcatgaacaatgaccatggtgacatccagcaaataagaaatagatgaaacactgggatccagcagtattctttgttccacaaaaatacttagtccccagttctccatagcagcatacggatgcttaggcacagctaaaagatctagttttggcaaggaatagggcactttaaagtagtcttcataaaattctattaatctctttgttatatggagagcatagtccccggatcctcttctgatagcatcaggtcttgcatataatcgtactacaaccccactcttggtggtagtttctctgtatgtgaagttgcaaattgcccaggctaaataatatgtggacatgagaggggtctgtgaaaagtgatccgtaacccatccatcttcctcaaacacggaagtttccactggcatattagataaagataaataggttgcttgatgcttgatgctgattttgaaagtagccttgtagattggctcatcaaaacaaggaaatgcctttctggcatgtgtaggcgaaaactgagtaacaccaaggaatctttagtggcatagcacagcagtgaaaagcacagacttggagtcagactgccacctattagctgtatgatcttgaccacataacacttgtgcctcagtttctcttctcttcaccaagccatgttctattattgatcccatctttcttctgtgtcttcaggttttatcttgccctttgctttctcctgcagcaaacaaacaggctctaatgtgataaggtaagcaagtttatatggacttttcttctgatgctctttg

SEQ ID NO: 15598 - RNA, 6389 nt, Homo sapiens
  source 1..6389: mol_type = other RNA
gctgggattacaggcatgagccactgtgcccagccctattttgtagttttaaatagctcatgttgctacctgagccccagttttctcatcagaatattagggctcacaacatttattatgtttttgtgatgagtcaaataaaacaaaatgtgtaacagttctttgagaaagcaatgcattttatcaatacatggcataaccttaataatagcctcacaagatattatacttataatatttgtaaataatactatcacaaaaatcttagtcctatgatataattgtcctggagataatataaaataatgcaagtttatgacccaactaaaatacatgttattgaaactcaagaatagacctagtattgtagatgttagtcttagaggttgagattgtgtattttagaaacttcaaagattatagaaaaattttaagaaaaaatgtgtaaaaatggggaaatctttttatttacgagttacctggaaatgtttaatactcaatgtgataaataatgttgtcctttctaattgaaactacttttttgtacacatattggcacagcaaattgctatggctggaggttggacactttcaacagttagttatttcatgcatacatataatttgtaaagccgacaaaaaagaaaagataaaaactctaagtagaaaatagaattttataactacgttttacagattattccaagagatatcattggttattttattcttttgaaaatattacttatttaaacaactaaaaaaaccggtaaagcctgatataatttcaacattagaaagaataaattattgaaaaatatgtagaacaaaaacaccatcttaatgccattggtaccactatactgttgagcaagtattatatgaggtattgaacattgcacataattatacacttaggatttgagattgtagataaaccagttgttcaaggccactaaaatactgaaaaaggattatgattattaacagtgaggaggaaaatacaactataaaagcccttcaaactcaaatctggaaatggtaattttactcaaaaatataccacaactactaagagattttagtaattcatgacacaaaacaagacatccacctctaatttttttcttatctattacatgaattcagtggtgatagaccacatatttgggacctccatcgcagtgtgatatttagtattgttatattttagaagttactcatttaattaaggattttataaacgtgatatgtggtaactggattttatcatttctgataaatggaaaaagtttagattttatactaaaagtattatcatgcctattcacatcatgtaaaatatttaaaattcatgtattttaattgaatgaagtgctgaaaaatttaggtatgactaataggtattacttgcttatatgataaaattcagttttaggtggtactttattctatagattcggaaatagctcctcttttctactaatttaaaataattctatggctctggttcttaaaatgtctaattattttcactattcagtgcgtactgttagaatatatttctttcaatgatttgtaagatttggtggagtgaaaaacctcaggaaaataagacgtgatttacaaacatttggctatgtagagtagttgcattggtattttatactggtaaacttaaaatatgctaattttgaagcatctaagcaacgtttggagagctggcctactgggtgagaataccatttaaaaacatttgtgttacacaacacacagccatgaaaatggctattcaaaattcccaggtagaacacagttgtcagtgccaaaagaaaagctttgtacattaacacaagaaaaggaacttttcatcttaagggatggcacaactggcacaaaaggtcattaaatgctaatagacccacttgaggtatgctcgcttaatggaggattagagcaaaacagacttaaaagaccaacatgcagagaatttttttaactctctggactactcagcataaggtaggaaaacaaacaagatggaaaataaactctttttcagcactaataattataagtttgcataattgtttcatgcaaaaggaactttgacagaaaacgatggcaaaatctataggcaagactgacacaggagaactggaatagtagtttatacaaaaattttgtttgtattcatcttcatgtagcagaatagaccactgttcaagaagtagatgaaaaattcataacagttgagaaatttagttaggacatagaaagaataatgttgagataaattccttgaagccttttgcaactgtccttaagtttataaaaagagataaattttctttgatctgaagacattctttgtacatgtgcagtgtacaacatactatatacatatggggcttccctatgtacatatacatatgcatacactatctatatgccttttaaaatgtatacacagctttaactcaaagaaaatgagttagcaacacagtaatcattgccagacaatccaagtgctgaaataagtgatgttcatcatgtcaagggctattttacctctcacattgcccaaaattgagaatatcatttctgtttttagtttttctttcattgcaatactgattgtcatatataatctttgtgcttttgcataatgcccatcctaggtgtaacacatattcacacacaacactggacgtttgaaataagcatgctggaacacaggcaggacaatatatccatgcacagatattctgaatatgtttttccaaattgactgtaacatcaacatgcatcactatcatatttggtcctgtacagcaaggaatgtacagctgaagcaatcatggctagtttcacttgcaagagtttctttagagaggaacacccagtagagaaacagaacagaatgaatgaaacaaataaaaaatatcccccaaaaccaaaaaataaaaactaaaaaaaaaattcctcccacacgttaacactgaaaatctggccattttctaggtagtacattttcctcattccacaaaaagcgtgtcttctcataaacttctgagttgaattgtttgtttataagatacatatattagtgtcttagagcttttcctaaccattggaaaagctcgtcttggtaaagcattttccagcgcacattggcttcgacagtttccacagctcgtgagaaagaagcagcagctaccccatcatagtttttcatgaagttcttgagctctttgagttcaccttcagtattaagaaattctgtgacaccactgatgagtttggaattcataaacaatgcttctccatacctggtatttaatatcttccatttatccctgaaaaacttccaggcaaggtctcgaccatgtggatttcgagctacatggattatgacatcaattgcatcttgatccagcaccacctcagaattcagtgacagatttagaagcctgtttaataaattcctgtcatcactgcaagttaaggcttccaataatattttcttctcagaaactgctgtggtggaatggaatttcatccatatgaattcccagacatcctcatccagtagtgacactcctgtacagtatacgatgtctctaacatttagtggtattctgttcctgttgctggaaatccaatctgaaataagtgttgatgcctgttggtgacagtgcttgttgccaaaactgcaggccagcattataacttctctacgtagttcttcatgttggtaggatgcttgaacaagagatccattaaaattatttttcggccacccaagcttgatatatgttgttgcaacttgctttaaaatatattcattgaaaatgttgtagttttccatgcggtccagtaatttatctagaggataaagagctcggctggcagcatgccaaggaagaaaatccttctcctcagacaggtatctgataatctccagaggaatattctgaggcaaatagccagccctggctaggctgaaggcatcatcgatcaagcccgctcggttactgacagaaagaacctcatgattccggattaattgatcaattaataatctccagttccttaggtcatagttgactctaaaatagccagtttgattgatgttccccagcagccagcttcctttgtccaaataagttattctgtggtgctctgatttgttagacacccaaataattgcttctgaagacacatggcttctatttcctaccacaatagttaatggaatctgccacaggtaactgttattctgaagtttaagtgctttagttttagcactgatatcatagataaaatgctgttgggtaattattattctattttctgctgttgtgtttcccaagatggtgataacaggataacccatctggagtgtccactgatccattacttcttgtatatttacatatttcccatttctttttaaagcctccgataatgtattccagagatcatttctggctgcattaccatacttatgaatggttaaataatcttgcaaacccctctggaaaactgaatggcccataaaattagccagcattcttattaaagcagcaccctttttatatgcgatccagtcaaacaccctgtcaatatctgttgcctgcagcacttcctgtgatactggatgggaactggccaaaccgtccagcagcatcacttcatgcagaacatcggtcagaaacctctgcttttccatgttccagccaggatagaggtagtctgtaccaacaaattcaaagtagtgagcaaacccttccttcagccacacgtcttcccaccacacaggcgtcacaaggtcaccaaaccactggtgacatatctcatgaacaatgaccatggtgacatccagcaaataagaaatagatgaaacactgggatccagcagtattctttgttccacaaaaatacttagtccccagttctccatagcagcatacggatgcttaggcacagctaaaagatcttctgaaaggccggaaggttctgcagaccccggggagaatagctgaaggcagctgtcctataaccctgaggcagacggcaaggagtaggtacaagggactgtgggggaatttatcttaaacaaggttgtttacttatattgaccaggaactgacctttgatcatctgcacatgtgacactgcctgaaaggggaacaataaatgttaattagctacaggttgtgttggctccaggttttcggcattgtgcctgcactgaataaaagcaagcagctccagcttcttggggctgttctctggccactagagccaggtagtcacctagctgctcttaaactgcatacccatgtatgagtactcatttcatctgtctgccagggtctgcgggacagacccagcagtccgccacacagtctctgtaatgctgttgctctctaatgcctccgatcaggcccagcaaaggagaaagggggtaagaaaggaagtctctataccatggcttatataaagcagaccacctgcaaatcaacgatggtaaagaacctaggaagcaactggctacaaaagtgaaccctctatgggaggaagaaagaaacctcatagttacaggcctggtactgtggcactccgtgaaatttgttatcagaagtccactgaacttctgattagcaaatttctcttccagcatctggtccaagaaattgctcagaacttcaaaacatctgtgcttcctgagagcagctattggagctttgcaggaagtgagacctatctggttgacctttttgaggacatcaacctgtgtgctatccatgtaaaacatgtaacaggtatgccaataaacagataataggccacatacatgaagtatatgcctaagaatccactatgatgaggaacatttcattctcaaaaaaaaaaaaacctcttcttcctgttattggcagatctgaacattaggtattttttccccatagaatcaaaaggtacctaaatataagattgtgagtggaaaaatagcagacagaaatcagatagtggcattttttccattttcatcatgtgaatttttaatgtaaatgtggggacataaagcattaatgtaagtcaaaatatttcagtgatcaagtttcagcagttcaacttcataacaaccacagataaacctgttaaatttttcttcacaatgtcagcatttggcttgtttttaaaataagtaaatttcttattaacagcaactaaatggtgtttgtggcattttttatcatacagtaaaaagtatagtacatccattgactatacttttctgagttgtcctacacacaagttcatgtttttaatgttgtctttcttgagtgctatttctgtaagtgtactattaaaataaa

SEQ ID NO: 15599 - RNA, 6383 nt, Homo sapiens
  source 1..6383: mol_type = other RNA
gctgggattacaggcatgagccactgtgcccagccctggctgtattcttgaagctgcccggggaaggctcacgaagggaggagcatctggttgtacctgattctggagacagcattttacctgcccctttacccactgtactccatccaaaatgaccctgcagtgccctgcagaggtctcaggccttggcctagagaacagagggctttgctcgtgctccccgctctgtctgcagtgctcttcctcttctatagccactcgaccatatctaggaatgcccagctcagtctacctctgaccctcacagtcctgttgacctgaggttctggatcagtgtccccacaaagcccagtcgtgttgccaagtgatgggtgtaggcgccagcactgtggcacttgctgagagtggcatatgattttttgcaggtcctagccctgggggtagcccagacacccccccagtgctgacaggttatgtgctgtggagggtgctgaaatggtttctcctccagtgggctggaatcacagatgggctgtttacggagcaagtgccggctccaccccatgagatctgggggttagagatgagcaggatgagtcctttgtaactgagaatgaagctgtacccctttctctccctgcagccctgaatcacttgctgggggtctggaggaggggttcacccttagggctgcttcatggtgggtgggctgactttgtggaaaaatgcccccacttcagccatgtttgtcttatcacggtgcagaaagatcacccaccatctctccttttccttcccagatgctccagaaaacctagatgagcagattaagaaagtgtcccagcagatccttgagaagcgagcctatatctgtgcccaccctctggacaggacatgctgaggcaggggacagtgtcccctgctaccgcccgcccctacccatggcccgttgctggatgactgttactcttttttcagaaggtgttgggattatcacaggttaagccttttgttccccgtctgcacctgaagggttgtcgcctggcctgggagagcctcttccaggttttgacctgcaggcagtgctctctaacaggaccatcacagcttctgaactgagccggagagagagaatggaattgctgacccctggaactggcgggtattctggtcattgaggagacaccatagtggaaactggggcttatgctgctgcctccagggtgtgaggtgggtggggacctgtgtcaggtgtggatagccatttctgctcaaccacacattctctaagaaacagcttgaaagctctgtctgggtcattcatttaaactagaagcagaggcacttaaaacatgtaccaggaaccatttaacaaagaatataaaatgtcacaatctgtgtactgttagcctttgctgtacttgtcacactgttccttagaaccagcctttaatgggtgacagcaggaccctgagaaccaccctttggtgatggcctcgggtcccctttgtcctcaccctgcaaggagggcccagaatgctaaggagcagacacacagtgcaggccacaatcccttggggttatgagcccttagtttttatccttctcaggagatgatggggaggctgtctcagctgatgatgttcccacctagggactttagtttctttacaagaactggcttctactcttgaggagaggatgaatggtatctccaggccagcaggcctttgcatttctccagcctcccttctgctggcacttgaaagattacaccaggtcccagcgtgctcactgtggtgaactttaagctttgatgtggtccttgggtggtctggagctctaaaatgcctattgtggacactcccttgagcacagagaaggcagccgactctttttcctccaagtatattcccaatttactgtgatgctggaaataggcaaggaggagactgggaacttggagagctgagctggctgagtggggctggcctgagcattctgccaggggtttggtaactagtttttaaaatggggaaagtttgtaaatattgtgaccgtgtaaataacctctcagtgaaacctgaagttctgttagtgatagcagggcagcattttgcacaaaatgaagcatgcatacctctggacagaaggctgcttagagtttctttgcacaggagaagtttggggaggggctgtcagacccaccccccttctgtgcagccttctggaagggggcttcactctaggctggtggcgtgtaaggcctcagtcttacatgccaatggagaatggcaagttctccattcatccatctgggttgaaaaggcctagcgaccagttcaagcctctccctctcatctgtagttgctaacttttcttaaacatgttgtgggaagaggagaccccagcaagtgtttcttaagtgatttcaccagtgaaacccccaggagacttttgctgggaaggctggcagtggagctcactaggaagccttcttaccaaggaaaagccttgtgttcttaggctagacagctctcctagctggagcctccttgagagccacagcagtaactgtgggcctgggacatgcccacagagagcaggtctcttcaggcaacctgggagatctagggcctactggggagggagggagccaagtctaggcaaatggagaaagtgacatttcagcaaacttgttagcacttccatggagctgtgatcagttgtccttaggagtcgaggaggagaggaagccatcacgttcacctgacctagttttctgggagaagtttctctggcagaccttgtttttagataggctcatgtctctttctccctgaacaaaggttctggctctgttaaccaagtttgggttctatgttaacctccagatgatcctgagatcaattttcataaacagggataaagaggaagaggacttggagggactggtacagcaagacctacgtttcctgtctctgccttaccccaaagaaagaactgtcagtatctttgccgctggaaggtcccagtgaagcccagagcctctgcccccagctcttggctggacacctagagatcagtcatgggtaatagtgttgaagctcaggaagcctttagacctgtcttccaacttccccactttatagccaagaaaccagacccagggcatgaagggatttgcctcaagtcacacaaatgtcacacttggggctagaatcctggtctgagttccagcccagcattcaatctcttttttcagacccattctgcatcttgcttttcttagcatagaaagtttggttgatagtgtaaacaaaatggataccactgaagatgcagagtggcacagagctcctgcctgcccacggcatcaggaggcccagcttggcaaacccttgcctgttacctgttacaggctttggtgcgggcgaagggagcagctcgaggaaaggtggtggtttcttgtacagatcaaagtccacgtggtgcctgtcccagctccacctgtctcgatccaacacaggctccagtacattagcaaacagggagttttccttccactcctcattcagctctttgatgggtggcagcttgagatcctgaaagctgctttcggtgtcgctctgaagacctgtcacttggaatcccctggctgtgagccaggcctggcgggatttcttctgggctttcttctcctcttccttcaagtccaggggctccaccatggctgagaggtaatcctgtgagtacgtgaatctctttcttggctccttggctatctcttgatacagctccttcttggcaagctctgtagaattcatggtctgggtactatagttgtagacggccttgttggcaggggctgaaattttaatcaccttcgccacggacttcggaggcttcttgctgacctggtaggcttctgtgatatttttctggatgaaactgtgctttttgtctttgttcttcataagcatggcactccgccactgcaggtacttctcctggtgggcgtggatctctaaggtgagggtggagttccgactgtggtagtcctcaagattgggggcaggctgaggtggtagggcaaacagtttctcatctgtgagttcttcttgcgaaaggggcatcccaaactcttggctcaagtcttttatcatagcagaggagggcagcaggtccctcaccgtcacgtcccagagggtggtgctgttatagcagatgtcgtggatcctggctagagcctggaagacccgcctccgctcagtgtctcgcaggaagaacaccgcctgctgcagcagcagctccgtgggctggaagaggtgcacgtggtacaggatggcctccaggtccccatagagccggctgcggaacagcagctgtgagttgtacagcaccttgtatttcctgtgttctgacctgggaatccagctttggtggttctcccacagctgcctcaagccttggtcggccaggccttccaggatgaaaaggtgtgtcttcccgtccagcaggtggaagccagtgagcacatccaggtgctgctgctcctggacccgcacacgcaccttgaaggctgacaggatctgctgcagggtcctgacagggtaggagtccaggccgagggccttagcgttgatcatggtgatgtcctgcagcaggctgtggagcagggagaccttcttaaagtcaaagacgaagatgatgcggccaaactgggagcccccaaggtcaggatcagcagctctggccccggccctcagtggcaccgcgatgtccactcgcaacttgagctgggagtcagcctctaggtagttgcccctgggcattgggccgtgctggtggccatctctggggaccccaagccccacaaccttccttctcctgctgtcctggccgcagtgtgtgggctgaacctcacagctgtggatggggacggccagattcaagtacttgtggccaaggaggaggtcagcaaaactgacctgggcgatgccataagggtaccacatcttgttctgggactcaaaggggttgttctctgtctctctgggagagatgagggcctggaagttgaggtatgaatccagagggtcctccccaaacagcacgggcttctgagaacactcctctgacttgcggtcccggtcgtgaacttccaccaccatgggggggccctccaggtattcccttaggtcactggggtgcagtgccccaaggaagatgacgttgatgtcctggaaataaacgtgggttccatggggctcccccttggtcttgtgaactggagtcttatggaactggtacttgcagtacacaggcatgcacagcctctctagttcctgaatgggtacaggctgtgatggaaggcaggaagcacacttgatctttatggtcaggggatttaaatcctgcttttgctcctcggtcatgatcggaacttctgtttttaaagtcaaaaggcaatctaaaatgttggcagacttctcactgccacgactcacgacagtttgccatccggcaaggagcggcatgacggccagctggatggagaaagcgctctgcttcctggggcctgtcagcgtggggtctgcctcttcttctgccaggggcttcttatgtctcctctggattttccttcttccctctgaatctttccctttaatttgagacctttgtctgtctaatatgtttgttaagctgctaagtgattcactctcaattaattccttgatctccatcatgcttgctcctgccaaagaaatggttggtgttcttgaaacactccattgaatcgtggaagaatcgtccattttgagggacttctcatattcctcactgttcttggaagaagtttcgggctctgcttggtgagaaccttgcaaagactttgggtgtttttctgttttttcttgttttcctggcggatgttcctggttcgactcttctctgacaatgttggtattctcaatgccctgttcagataattttctctgatttaaaaccaaatgtctcacttccatattcacagggaaggccagtgagatggtgaatttgcaggggaccacgtggggcacgtcggagctgaaagtgctggcaggctcagatgaggactcgatgctgctgcacgggcggtcagagtcagactcctgggccctggccttggccttcaggtgttcctccacgtcacactcgctcgtggactggtaaaagctagtgatggaggagatgggctctatgcttgcggggtcctcttcccactcccaggcatgtagcgacatgctgcagagcgcactgctggccgccggcgctcctgctgacatacctcctctgccaagaagctcactgccttccacagcacatccatcattcttcat

SEQ ID NO: 15600 - RNA, 6060 nt, Homo sapiens
  source 1..6060: mol_type = other RNA
gctgggattacaggcatgagccactgtgcccagccctggctgtattcttgaagctgcccggggaaggctcacgaagggaggagcatctggttgtacctgattctggagacagcattttacctgcccctttacccactgtactccatccaaaatgaccctgcagtgccctgcagaggtctcaggccttggcctagagaacagagggctttgctcgtgctccccgctctgtctgcagtgctcttcctcttctatagccactcgaccatatctaggaatgcccagctcagtctacctctgaccctcacagtcctgttgacctgaggttctggatcagtgtccccacaaagcccagtcgtgttgccaagtgatgggtgtaggcgccagcactgtggcacttgctgagagtggcatatgattttttgcaggtcctagccctgggggtagcccagacacccccccagtgctgacaggttatgtgctgtggagggtgctgaaatggtttctcctccagtgggctggaatcacagatgggctgtttacggagcaagtgccggctccaccccatgagatctgggggttagagatgagcaggatgagtcctttgtaactgagaatgaagctgtacccctttctctccctgcagccctgaatcacttgctgggggtctggaggaggggttcacccttagggctgcttcatggtgggtgggctgactttgtggaaaaatgcccccacttcagccatgtttgtcttatcacggtgcagaaagatcacccaccatctctccttttccttcccagatgctccagaaaacctagatgagcagattaagaaagtgtcccagcagatccttgagaagcgagcctatatctgtgcccaccctctggacaggacatgctgaggcaggggacagtgtcccctgctaccgcccgcccctacccatggcccgttgctggatgactgttactcttttttcagaaggtgttgggattatcacaggttaagccttttgttccccgtctgcacctgaagggttgtcgcctggcctgggagagcctcttccaggttttgacctgcaggcagtgctctctaacaggaccatcacagcttctgaactgagccggagagagagaatggaattgctgacccctggaactggcgggtattctggtcattgaggagacaccatagtggaaactggggcttatgctgctgcctccagggtgtgaggtgggtggggacctgtgtcaggtgtggatagccatttctgctcaaccacacattctctaagaaacagcttgaaagctctgtctgggtcattcatttaaactagaagcagaggcacttaaaacatgtaccaggaaccatttaacaaagaatataaaatgtcacaatctgtgtactgttagcctttgctgtacttgtcacactgttccttagaaccagcctttaatgggtgacagcaggaccctgagaaccaccctttggtgatggcctcgggtcccctttgtcctcaccctgcaaggagggcccagaatgctaaggagcagacacacagtgcaggccacaatcccttggggttatgagcccttagtttttatccttctcaggagatgatggggaggctgtctcagctgatgatgttcccacctagggactttagtttctttacaagaactggcttctactcttgaggagaggatgaatggtatctccaggccagcaggcctttgcatttctccagcctcccttctgctggcacttgaaagattacaccaggtcccagcgtgctcactgtggtgaactttaagctttgatgtggtccttgggtggtctggagctctaaaatgcctattgtggacactcccttgagcacagagaaggcagccgactctttttcctccaagtatattcccaatttactgtgatgctggaaataggcaaggaggagactgggaacttggagagctgagctggctgagtggggctggcctgagcattctgccaggggtttggtaactagtttttaaaatggggaaagtttgtaaatattgtgaccgtgtaaataacctctcagtgaaacctgaagttctgttagtgatagcagggcagcattttgcacaaaatgaagcatgcatacctctggacagaaggctgcttagagtttctttgcacaggagaagtttggggaggggctgtcagacccaccccccttctgtgcagccttctggaagggggcttcactctaggctggtggcgtgtaaggcctcagtcttacatgccaatggagaatggcaagttctccattcatccatctgggttgaaaaggcctagcgaccagttcaagcctctccctctcatctgtagttgctaacttttcttaaacatgttgtgggaagaggagaccccagcaagtgtttcttaagtgatttcaccagtgaaacccccaggagacttttgctgggaaggctggcagtggagctcactaggaagccttcttaccaaggaaaagccttgtgttcttaggctagacagctctcctagctggagcctccttgagagccacagcagtaactgtgggcctgggacatgcccacagagagcaggtctcttcaggcaacctgggagatctagggcctactggggagggagggagccaagtctaggcaaatggagaaagtgacatttcagcaaacttgttagcacttccatggagctgtgatcagttgtccttaggagtcgaggaggagaggaagccatcacgttcacctgacctagttttctgggagaagtttctctggcagaccttgtttttagataggctcatgtctctttctccctgaacaaaggttctggctctgttaaccaagtttgggttctatgttaacctccagatgatcctgagatcaattttcataaacagggataaagaggaagaggacttggagggactggtacagcaagacctacgtttcctgtctctgccttaccccaaagaaagaactgtcagtatctttgccgctggaaggtcccagtgaagcccagagcctctgcccccagctcttggctggacacctagagatcagtcatgggtaatagtgttgaagctcaggaagcctttagacctgtcttccaacttccccactttatagccaagaaaccagacccagggcatgaagggatttgcctcaagtcacacaaatgtcacacttggggctagaatcctggtctgagttccagcccagcattcaatctcttttttcagacccattctgcatcttgcttttcttagcatagaaagtttggttgatagtgtaaacaaaatggataccactgaagatgcagagtggcacagagctcctgcctgcccacggcatcaggaggcccagcttggcaaacccttgcctgttacctgttacaggctttggtgcgggcgaagggagcagctcgaggaaaggtggtggtttcttgtacagatcaaagtccacgtggtgcctgtcccagctccacctgtctcgatccaacacaggctccagtacattagcaaacagggagttttccttccactcctcattcagctctttgatgggtggcagcttgagatcctgaaagctgctttcggtgtcgctctgaagacctgtcacttggaatcccctggctgtgagccaggcctggcgggatttcttctgggctttcttctcctcttccttcaagtccaggggctccaccatggctgagaggtaatcctgtgagtacgtgaatctctttcttggctccttggctatctcttgatacagctccttcttggcaagctctgtagaattcatggtctgggtactatagttgtagacggccttgttggcaggggctgaaattttaatcaccttcgccacggacttcggaggcttcttgctgacctggtaggcttctgtgatatttttctggatgaaactgtgctttttgtctttgttcttcataagcatggcactccgccactgcaggtacttctcctggtgggcgtggatctctaaggtgagggtggagttccgactgtggtagtcctcaagattgggggcaggctgaggtggtagggcaaacagtttctcatctgtgagttcttcttgcgaaaggggcatcccaaactcttggctcaagtcttttatcatagcagaggagggcagcaggtccctcaccgtcacgtcccagagggtggtgctgttatagcagatgtcgtggatcctggctagagcctggaagacccgcctccgctcagtgtctcgcaggaagaacaccgcctgctgcagcagcagctccgtgggctggaagaggtgcacgtggtacaggatggcctccaggtccccatagagccggctgcggaacagcagctgtgagttgtacagcaccttgtatttcctgtgttctgacctgggaatccagctttggtggttctcccacagctgcctcaagccttggtcggccaggccttccaggatgaaaaggtgtgtcttcccgtccagcaggtggaagccagtgagcacatccaggtgctgctgctcctggacccgcacacgcaccttgaaggctgacaggatctgctgcagggtcctgacagggtaggagtccaggccgagggccttagcgttgatcatggtgatgtcctgcagcaggctgtggagcagggagaccttcttaaagtcaaagacgaagatgatgcggccaaactgggagcccccaaggtcaggatcagcagctctggccccggccctcagtggcaccgcgatgtccactcgcaacttgagctgggagtcagcctctaggtagttgcccctgggcattgggccgtgctggtggccatctctggggaccccaagccccacaaccttccttctcctgctgtcctggccgcagtgtgtgggctgaacctcacagctgtggatggggacggccagattcaagtacttgtggccaaggaggaggtcagcaaaactgacctgggcgatgccataagggtaccacatcttgttctgggactcaaaggggttgttctctgtctctctgggagagatgagggcctggaagttgaggtatgaatccagagggtcctccccaaacagcacgggcttctgagaacactcctctgacttgcggtcccggtcgtgaacttccaccaccatgggggggccctccaggtattcccttaggtcactggggtgcagtgccccaaggaagatgacgttgatgtcctggaaataaacgtgggttccatggggctcccccttggtcttgtgaactggagtcttatggaactggtacttgcagtacacaggcatgcacagcctctctagttcctgaatgggtacaggctgtgatggaaggcaggaagcacacttgatctttatggtcaggggatttaaatcctgcttttgctcctcggtcatgatcggaacttctgtttttaaagtcaaaaggcaatctaaaatgttggcagacttctcactgccacgactcacgacagtttgccatccggcaaggagcggcatgacggccagctggatggagaaagcgctctgcttcctggggcctgtcagcgtggggtctgcctcttcttctgccaggggcttcttatgtctcctctggattttccttcttccctctgaatctttccctttaatttgagacctttgtctgtctaatatgtttgttaagctgctaagtgattcactctcaattaattccttgatctccatcatgcttgctcctgccaaagaaatggttggtgttcttgaaacactccattgaatcgtggaagaatcgtccattttgagggacttctcatattcctcactgttcttggaagaagtttcgggctctgcttggtgagaaccttgcaaagactttgggtgtttttctgttttttcttgttttcctggcggatgttcctggttcgactcttctctgacaatgttggtattctcaatgccctgttcagataattttctctgatttaaaaccaaatgtctcacttccgtggtcccagctactcaggaggctgaggcagga

SEQ ID NO: 15601 - RNA, 12103 nt, Homo sapiens
  source 1..12103: mol_type = other RNA
gctgggattacaggcatgagccactgtgcccagccctggctgtattcttgaagctgcccggggaaggctcacgaagggaggagcatctggttgtacctgattctggagacagcattttacctgcccctttacccactgtactccatccaaaatgaccctgcagtgccctgcagaggtctcaggccttggcctagagaacagagggctttgctcgtgctccccgctctgtctgcagtgctcttcctcttctatagccactcgaccatatctaggaatgcccagctcagtctacctctgaccctcacagtcctgttgacctgaggttctggatcagtgtccccacaaagcccagtcgtgttgccaagtgatgggtgtaggcgccagcactgtggcacttgctgagagtggcatatgattttttgcaggtcctagccctgggggtagcccagacacccccccagtgctgacaggttatgtgctgtggagggtgctgaaatggtttctcctccagtgggctggaatcacagatgggctgtttacggagcaagtgccggctccaccccatgagatctgggggttagagatgagcaggatgagtcctttgtaactgagaatgaagctgtacccctttctctccctgcagccctgaatcacttgctgggggtctggaggaggggttcacccttagggctgcttcatggtgggtgggctgactttgtggaaaaatgcccccacttcagccatgtttgtcttatcacggtgcagaaagatcacccaccatctctccttttccttcccagatgctccagaaaacctagatgagcagattaagaaagtgtcccagcagatccttgagaagcgagcctatatctgtgcccaccctctggacaggacatgctgaggcaggggacagtgtcccctgctaccgcccgcccctacccatggcccgttgctggatgactgttactcttttttcagaaggtgttgggattatcacaggttaagccttttgttccccgtctgcacctgaagggttgtcgcctggcctgggagagcctcttccaggttttgacctgcaggcagtgctctctaacaggaccatcacagcttctgaactgagccggagagagagaatggaattgctgacccctggaactggcgggtattctggtcattgaggagacaccatagtggaaactggggcttatgctgctgcctccagggtgtgaggtgggtggggacctgtgtcaggtgtggatagccatttctgctcaaccacacattctctaagaaacagcttgaaagctctgtctgggtcattcatttaaactagaagcagaggcacttaaaacatgtaccaggaaccatttaacaaagaatataaaatgtcacaatctgtgtactgttagcctttgctgtacttgtcacactgttccttagaaccagcctttaatgggtgacagcaggaccctgagaaccaccctttggtgatggcctcgggtcccctttgtcctcaccctgcaaggagggcccagaatgctaaggagcagacacacagtgcaggccacaatcccttggggttatgagcccttagtttttatccttctcaggagatgatggggaggctgtctcagctgatgatgttcccacctagggactttagtttctttacaagaactggcttctactcttgaggagaggatgaatggtatctccaggccagcaggcctttgcatttctccagcctcccttctgctggcacttgaaagattacaccaggtcccagcgtgctcactgtggtgaactttaagctttgatgtggtccttgggtggtctggagctctaaaatgcctattgtggacactcccttgagcacagagaaggcagccgactctttttcctccaagtatattcccaatttactgtgatgctggaaataggcaaggaggagactgggaacttggagagctgagctggctgagtggggctggcctgagcattctgccaggggtttggtaactagtttttaaaatggggaaagtttgtaaatattgtgaccgtgtaaataacctctcagtgaaacctgaagttctgttagtgatagcagggcagcattttgcacaaaatgaagcatgcatacctctggacagaaggctgcttagagtttctttgcacaggagaagtttggggaggggctgtcagacccaccccccttctgtgcagccttctggaagggggcttcactctaggctggtggcgtgtaaggcctcagtcttacatgccaatggagaatggcaagttctccattcatccatctgggttgaaaaggcctagcgaccagttcaagcctctccctctcatctgtagttgctaacttttcttaaacatgttgtgggaagaggagaccccagcaagtgtttcttaagtgatttcaccagtgaaacccccaggagacttttgctgggaaggctggcagtggagctcactaggaagccttcttaccaaggaaaagccttgtgttcttaggctagacagctctcctagctggagcctccttgagagccacagcagtaactgtgggcctgggacatgcccacagagagcaggtctcttcaggcaacctgggagatctagggcctactggggagggagggagccaagtctaggcaaatggagaaagtgacatttcagcaaacttgttagcacttccatggagctgtgatcagttgtccttaggagtcgaggaggagaggaagccatcacgttcacctgacctagttttctgggagaagtttctctggcagaccttgtttttagataggctcatgtctctttctccctgaacaaaggttctggctctgttaaccaagtttgggttctatgttaacctccagatgatcctgagatcaattttcataaacagggataaagaggaagaggacttggagggactggtacagcaagacctacgtttcctgtctctgccttaccccaaagaaagaactgtcagtatctttgccgctggaaggtcccagtgaagcccagagcctctgcccccagctcttggctggacacctagagatcagtcatgggtaatagtgttgaagctcaggaagcctttagacctgtcttccaacttccccactttatagccaagaaaccagacccagggcatgaagggatttgcctcaagtcacacaaatgtcacacttggggctagaatcctggtctgagttccagcccagcattcaatctcttttttcagacccattctgcatcttgcttttcttagcatagaaagtttggttgatagtgtaaacaaaatggataccactgaagatgcagagtggcacagagctcctgcctgcccacggcatcaggaggcccagcttggcaaacccttgcctgttacctgttacaggctttggtgcgggcgaagggagcagctcgaggaaaggtggtggtttcttgtacagatcaaagtccacgtggtgcctgtcccagctccacctgtctcgatccaacacaggctccagtacattagcaaacagggagttttccttccactcctcattcagctctttgatgggtggcagcttgagatcctgaaagctgctttcggtgtcgctctgaagacctgtcacttggaatcccctggctgtgagccaggcctggcgggatttcttctgggctttcttctcctcttccttcaagtccaggggctccaccatggctgagaggtaatcctgtgagtacgtgaatctctttcttggctccttggctatctcttgatacagctccttcttggcaagctctgtagaattcatggtctgggtactatagttgtagacggccttgttggcaggggctgaaattttaatcaccttcgccacggacttcggaggcttcttgctgacctggtaggcttctgtgatatttttctggatgaaactgtgctttttgtctttgttcttcataagcatggcactccgccactgcaggtacttctcctggtgggcgtggatctctaaggtgagggtggagttccgactgtggtagtcctcaagattgggggcaggctgaggtggtagggcaaacagtttctcatctgtgagttcttcttgcgaaaggggcatcccaaactcttggctcaagtcttttatcatagcagaggagggcagcaggtccctcaccgtcacgtcccagagggtggtgctgttatagcagatgtcgtggatcctggctagagcctggaagacccgcctccgctcagtgtctcgcaggaagaacaccgcctgctgcagcagcagctccgtgggctggaagaggtgcacgtggtacaggatggcctccaggtccccatagagccggctgcggaacagcagctgtgagttgtacagcaccttgtatttcctgtgttctgacctgggaatccagctttggtggttctcccacagctgcctcaagccttggtcggccaggccttccaggatgaaaaggtgtgtcttcccgtccagcaggtggaagccagtgagcacatccaggtgctgctgctcctggacccgcacacgcaccttgaaggctgacaggatctgctgcagggtcctgacagggtaggagtccaggccgagggccttagcgttgatcatggtgatgtcctgcagcaggctgtggagcagggagaccttcttaaagtcaaagacgaagatgatgcggccaaactgggagcccccaaggtcaggatcagcagctctggccccggccctcagtggcaccgcgatgtccactcgcaacttgagctgggagtcagcctctaggtagttgcccctgggcattgggccgtgctggtggccatctctggggaccccaagccccacaaccttccttctcctgctgtcctggccgcagtgtgtgggctgaacctcacagctgtggatggggacggccagattcaagtacttgtggccaaggaggaggtcagcaaaactgacctgggcgatgccataagggtaccacatcttgttctgggactcaaaggggttgttctctgtctctctgggagagatgagggcctggaagttgaggtatgaatccagagggtcctccccaaacagcacgggcttctgagaacactcctctgacttgcggtcccggtcgtgaacttccaccaccatgggggggccctccaggtattcccttaggtcactggggtgcagtgccccaaggaagatgacgttgatgtcctggaaataaacgtgggttccatggggctcccccttggtcttgtgaactggagtcttatggaactggtacttgcagtacacaggcatgcacagcctctctagttcctgaatgggtacaggctgtgatggaaggcaggaagcacacttgatctttatggtcaggggatttaaatcctgcttttgctcctcggtcatgatcggaacttctgtttttaaagtcaaaaggcaatctaaaatgttggcagacttctcactgccacgactcacgacagtttgccatccggcaaggagcggcatgacggccagctggatggagaaagcgctctgcttcctggggcctgtcagcgtggggtctgcctcttcttctgccaggggcttcttatgtctcctctggattttccttcttccctctgaatctttccctttaatttgagacctttgtctgtctaatatgtttgttaagctgctaagtgattcactctcaattaattccttgatctccatcatgcttgctcctgccaaagaaatggttggtgttcttgaaacactccattgaatcgtggaagaatcgtccattttgagggacttctcatattcctcactgttcttggaagaagtttcgggctctgcttggtgagaaccttgcaaagactttgggtgtttttctgttttttcttgttttcctggcggatgttcctggttcgactcttctctgacaatgttggtattctcaatgccctgttcagataattttctctgatttaaaaccaaatgtctcacttctgacttatgaaaagctcccacgtcgtctgtgaagccggcagtctttaatcggtaatatctgacttttcttgacatcttgtctttagtgttccagagcctcaaggtgattttgtggaaatttattttctttaataattcctttgtcacagtgatattaaaagtctgctcccacgacacccaggctttgtcaccttcgtgccacggcttcacagtccatattcacagggaaggccagtgagatggtgaatttgcaggggaccacgtggggcacgtcggagctgaaagtgctggcaggctcagatgaggactcgatgctgctgcacgggcggtcagagtcagactcctgggccctggccttggccttcaggtgttcctccacgtcacactcgctcgtggactggtaaaagctagtgatggaggagatgggctctatgcttgcggggtcctcttcccactcccaggcatgtagcgacatgctgcagagcgcactgctggccgccggcgctcctgcgagcggatgcgctgggcggcagcggggagttggaccgcggcggcaactcccgtaccggatccacagccacctgggcgaagagactccaagactgagaggagcgtccgccggtgcagggagggccgcaggcccagccactcagctacgtttggcggttgctaggagacgcgagggcgtgcggcctgggggcggggctccgcggggcggggctttccccctcagccactgcgcgcagtttgtcaaatggctacatccaggttcagaaaccagctgccttcattccttcactcatgcattcactcattaaggagtttctactcggaacgtcagcacctactataagcctggtccttgcccgtacgatgggaggtaggggttgatggctccttcctccccctccatcagctcccacctcccattctttaataaaagcaaaggaagctgtgggctctgcaaactccagacctccccacgatccctctcattagattctctgcttctgtcgccgatgtccttaaaaaccagacctccccacgatccctctcattagattctctgcttctgtcgctgatgtccttaaaatagcatgagaattcttgttagtgatcatgagcgccaactcagagatcagaaaacaaagcttagagaggtgaagcgattcgcccgaggtcacacagcaagtagggcgcagcactgtgttgaaatccggactgcctgactccaaagcctccgctcgtctgctaaaccacccaagctgagagccctggctgcggctcctaatgtagaggacctcagcacagcaagcggctgggacagagggctggggtaggcctcatggaggaagtgagcaacgccaaatctggggggtgactaggcagaggcggtgaaagcaagagaaagcatcccaggtagaggaacagcatatgcaaaggcccatagaggtgaaagggcatggcaagtttcaggaatgggtggcgaggctgtagcagtgtgcagggcccatggtacatagccccacagggcaggttagggcacaggactatgggcaatggggagccaaggcaggtcttctgttgagggagggcaccctgctccggcagtcagtttgttcaagagaatgggagctgaggctacacacaagcttggctattaagaaaactttagctgagttgagctatgacctactttgtgtcaaagagcaaaactgtggcgcagctggggctgagacccaagtcctgagcctcccagtgcatgcctccccagaccgctctcagggcatgggacagcccctttaatactgggtgctccaatactcctcgggttcagtctgaaaaacagcctcaagtacagctgttagggaagacaccaaatggcagtgggccctgtgaggagtgggttcaaactcttagcacgagaacggcaaccaccttgcccacaccccacctgcagcagcctggagactgctgtctgtatgccaggaagtgctcaggagacacatgaagggctggaagaatacaaagctactcagatacaccagcccccaaaagggccctttaacaagggcagttcaacactaccaccactcttggacagacatcaggcctcctgctccccaggtcctacccactggcctgaggctggtttccctccaaaggttcctagatcacatcaccacctaggacagaagccaatctcttcccaagctcaatagtgagaggccagaggtcttggaccaagggccaatgtgccatcctggatgtgcactggaaacacctacatgtcaaaaatacaattctgaggcttcattaaagacctgtggaagtgactctccaggggtggagcttagaaaccagtggcagattgtattttccaaagacagccacctcaaaagatcccctcccacataatcttccggcaggcattgtgaggttcacattcctcccacccagttggggggtctagtctccttctctggaaactgggcagacctctgtgactggctcagtcaaaagagtgcagaggaaatgacactatgtgatttctgaggccaggtcatataaattccatctacctctgccctgttcttttgaggtatagtattcatgctaggaatccagctagcatgttgtgaggaagcccaagcagccatgtgaaatggccacatgaaactgttgtgactgacggttcccagccaattgcagcctcaacccccagacatatgagagtgcaagacttcaaatgatcccagccctcagtctttgagccaccctggctgacattgaggaacagaaacaagctgtctccatcatgagaaattgtagatttataagcaaattgttgctctcttaaaccactaagttttggggtgatttgttgtgcaataaataataggaacgggagccatatttttaaattaccaccaagattgtattgcacaaccagaatatggaaccactgccctgagagagatggtgtctgggtcaagacctagggcatcacaggatgaagtgagggcaaaggtgtgctacccactactcaggtatgagacagtggtgggtctacaaccctacctcagtgaagatggcttcagggctggcagatcagaagcaaaggaaggggggcttctgtttcagttatctgttactgagtaaaaaccatccccaaacttaatggtgtcaaacaaacacttgttatttctcaccactccatgcatcagctgagtagttctctgctggcctcgcctgggctcactccctatgctgtgctcagctggaggaccaacatggctggaagctgccagaagtcctcacttgcatgtctggcagttgctgctggctcttcgtgggcccgctggttcccctccatgggttcccccgcccccagtggtacaccagcttccttctatgtggtgcctcatctcctcatagcccggcctggcttcctcagatggcattctcagagcagggatcccagagggcaaagaagaagttgcaaggcctcttgggacctaggcgtggaaccagcaccatgtcactctgctacatgccattaaccaaagcaagtcatgaggctggccccacttcaaggggatgaagacatggactgtacatctggtaagcagagggacaagcatccaggggcaggaggtgttcaaggtcactgaacaatccatcccttcatccttactctgccgggtggagggttcccaagctcccacaggctatgtagaggccttcctgaagctatcccaagactctggcagctggaagcatattgggaatcagctacatacaccttcttcttgccccttccccatttttaacagctttattgaagtattttttatttaataaaatccatccatttcaagcgtagaattcaatgattttcagtaactttacctagtgctgtaatcatcatcataaattcattttagaacattttcatccccctaataagacttcatgcacatttataattaatctctgttccaactcccagtcctaggcaaccatatctactttgtttctaaaaattggccttttctagacatttcctataaattgagtcagacactgtgttctggctttgtgactggtttctttcacctaccgttatgtttccaaggtttatttatgttgaggcatgtgtcagtatttcattccttttcatgactgaataatattctattgtatggacagaccacagtttgcctatccattcatcagttaatgggcatttggcttgggcatttagacatttatgaacaacgttgctatgaacattcccacacaagtctttgtgtggatgtgttttcatctctcttgggtcgatatctaggagtggaagagttgggtcgtatggtcattttgtgattaacttcttgagaaactgccaaactatcttccacaggggctgcatcattttgtgttcccatcaacaacatgaagtttcctgtttctccaaattcttgacaagatttattgcctgttttattcactacagctattctcatgagtataatatagtatttcatcatagttttcatgtgcatttccctaacaagaatactgagattgttttatgcacatgttggctatttatacaacttctttggtgaaatgtctgtttgtatcttcacccactttttgattggattgtttgtcttcttgttactgagttgttaagagttcattgtaaattcggaatataagtcctttactgggcatatgttttacaaatattttctcctagtctcttgttcgtcatattttcttaatagtgtcttttgaagtgcaaatgttttgaactttgatgaaggtccgattcatcatttttttcttttttggatcatgcatttggtgtcgtatctaagaaatctttgactaacaacaggcctatttttaatagaagtaaagcttggtgtctgaacactaagcaaatctactaaccaagacccctaaaaacccaaaagctttatgacactgaaaataatggcccaaggacattcccagacagttctgggctctggatagaacaacacaagtttccaaaaaacaggctgataataccacaagcttataaaatatgtatactccttggcccagtaataaatcactcaagatatggcacaaactgttcacagtatggtttttgcggagaaaagctgaaaaccacctcagtgggcatctgtgggggatgacaaagcaccttatagttcatccccagggagcacagagcagcctctggagcagtgtctgcaaagaaaccacagccaagctgtttacaaagctcagttcctgtgcaaagaaagatcccaatggcgccctttccactgtgcttttcatgtcaagttgaatgagctacgatttgcacactgtaaaattcagatgtacacagtcatgcaaccactacaccatgaagatagagtatttcaatcactccaaaaagttctttcatgcccaaatacatagaaaagtctggaaataaatacatcagaaatacacagtgatcctctcttggtggcagaatggtggatgatttttgctttttagcattttcccggacctttaaaagacactttaaacaatatactatttgaaatggctcaaacaatactgaactgacttcagaaaatcatttctttgccacagccctgactctctcccacacagacacacgcccatccccccagctcatacaaaagaacgcaaggagacctctgagtttgctcactttgaaccttaaacaaaaaccttgtggatgcaaccagaattatttcagaggtgcctggtaacaccgcagggcagacagacaggcctgacagcaaaccattatcaacccttacttccctgagctgtaggggagtggaggccggcaacggctcccagcaagacatttaaaagctttcttttcaatattgactggcccaggaaagctactgttcaaaggattccttcaccagctgcagggatggggggtggggagggtgttgcactcttgcctgggctaccagctcttagggctgacatgaaataaaatcaggttctttttttttttttttttt

SEQ ID NO: 15602 - RNA, 6283 nt, Homo sapiens
  source 1..6283: mol_type = other RNA
gctgggattacaggcatgagccactgtgcccagccctggctgtattcttgaagctgcccggggaaggctcacgaagggaggagcatctggttgtacctgattctggagacagcattttacctgcccctttacccactgtactccatccaaaatgaccctgcagtgccctgcagaggtctcaggccttggcctagagaacagagggctttgctcgtgctccccgctctgtctgcagtgctcttcctcttctatagccactcgaccatatctaggaatgcccagctcagtctacctctgaccctcacagtcctgttgacctgaggttctggatcagtgtccccacaaagcccagtcgtgttgccaagtgatgggtgtaggcgccagcactgtggcacttgctgagagtggcatatgattttttgcaggtcctagccctgggggtagcccagacacccccccagtgctgacaggttatgtgctgtggagggtgctgaaatggtttctcctccagtgggctggaatcacagatgggctgtttacggagcaagtgccggctccaccccatgagatctgggggttagagatgagcaggatgagtcctttgtaactgagaatgaagctgtacccctttctctccctgcagccctgaatcacttgctgggggtctggaggaggggttcacccttagggctgcttcatggtgggtgggctgactttgtggaaaaatgcccccacttcagccatgtttgtcttatcacggtgcagaaagatcacccaccatctctccttttccttcccagatgctccagaaaacctagatgagcagattaagaaagtgtcccagcagatccttgagaagcgagcctatatctgtgcccaccctctggacaggacatgctgaggcaggggacagtgtcccctgctaccgcccgcccctacccatggcccgttgctggatgactgttactcttttttcagaaggtgttgggattatcacaggttaagccttttgttccccgtctgcacctgaagggttgtcgcctggcctgggagagcctcttccaggttttgacctgcaggcagtgctctctaacaggaccatcacagcttctgaactgagccggagagagagaatggaattgctgacccctggaactggcgggtattctggtcattgaggagacaccatagtggaaactggggcttatgctgctgcctccagggtgtgaggtgggtggggacctgtgtcaggtgtggatagccatttctgctcaaccacacattctctaagaaacagcttgaaagctctgtctgggtcattcatttaaactagaagcagaggcacttaaaacatgtaccaggaaccatttaacaaagaatataaaatgtcacaatctgtgtactgttagcctttgctgtacttgtcacactgttccttagaaccagcctttaatgggtgacagcaggaccctgagaaccaccctttggtgatggcctcgggtcccctttgtcctcaccctgcaaggagggcccagaatgctaaggagcagacacacagtgcaggccacaatcccttggggttatgagcccttagtttttatccttctcaggagatgatggggaggctgtctcagctgatgatgttcccacctagggactttagtttctttacaagaactggcttctactcttgaggagaggatgaatggtatctccaggccagcaggcctttgcatttctccagcctcccttctgctggcacttgaaagattacaccaggtcccagcgtgctcactgtggtgaactttaagctttgatgtggtccttgggtggtctggagctctaaaatgcctattgtggacactcccttgagcacagagaaggcagccgactctttttcctccaagtatattcccaatttactgtgatgctggaaataggcaaggaggagactgggaacttggagagctgagctggctgagtggggctggcctgagcattctgccaggggtttggtaactagtttttaaaatggggaaagtttgtaaatattgtgaccgtgtaaataacctctcagtgaaacctgaagttctgttagtgatagcagggcagcattttgcacaaaatgaagcatgcatacctctggacagaaggctgcttagagtttctttgcacaggagaagtttggggaggggctgtcagacccaccccccttctgtgcagccttctggaagggggcttcactctaggctggtggcgtgtaaggcctcagtcttacatgccaatggagaatggcaagttctccattcatccatctgggttgaaaaggcctagcgaccagttcaagcctctccctctcatctgtagttgctaacttttcttaaacatgttgtgggaagaggagaccccagcaagtgtttcttaagtgatttcaccagtgaaacccccaggagacttttgctgggaaggctggcagtggagctcactaggaagccttcttaccaaggaaaagccttgtgttcttaggctagacagctctcctagctggagcctccttgagagccacagcagtaactgtgggcctgggacatgcccacagagagcaggtctcttcaggcaacctgggagatctagggcctactggggagggagggagccaagtctaggcaaatggagaaagtgacatttcagcaaacttgttagcacttccatggagctgtgatcagttgtccttaggagtcgaggaggagaggaagccatcacgttcacctgacctagttttctgggagaagtttctctggcagaccttgtttttagataggctcatgtctctttctccctgaacaaaggttctggctctgttaaccaagtttgggttctatgttaacctccagatgatcctgagatcaattttcataaacagggataaagaggaagaggacttggagggactggtacagcaagacctacgtttcctgtctctgccttaccccaaagaaagaactgtcagtatctttgccgctggaaggtcccagtgaagcccagagcctctgcccccagctcttggctggacacctagagatcagtcatgggtaatagtgttgaagctcaggaagcctttagacctgtcttccaacttccccactttatagccaagaaaccagacccagggcatgaagggatttgcctcaagtcacacaaatgtcacacttggggctagaatcctggtctgagttccagcccagcattcaatctcttttttcagacccattctgcatcttgcttttcttagcatagaaagtttggttgatagtgtaaacaaaatggataccactgaagatgcagagtggcacagagctcctgcctgcccacggcatcaggaggcccagcttggcaaacccttgcctgttacctgttacaggctttggtgcgggcgaagggagcagctcgaggaaaggtggtggtttcttgtacagatcaaagtccacgtggtgcctgtcccagctccacctgtctcgatccaacacaggctccagtacattagcaaacagggagttttccttccactcctcattcagctctttgatgggtggcagcttgagatcctgaaagctgctttcggtgtcgctctgaagacctgtcacttggaatcccctggctgtgagccaggcctggcgggatttcttctgggctttcttctcctcttccttcaagtccaggggctccaccatggctgagaggtaatcctgtgagtacgtgaatctctttcttggctccttggctatctcttgatacagctccttcttggcaagctctgtagaattcatggtctgggtactatagttgtagacggccttgttggcaggggctgaaattttaatcaccttcgccacggacttcggaggcttcttgctgacctggtaggcttctgtgatatttttctggatgaaactgtgctttttgtctttgttcttcataagcatggcactccgccactgcaggtacttctcctggtgggcgtggatctctaaggtgagggtggagttccgactgtggtagtcctcaagattgggggcaggctgaggtggtagggcaaacagtttctcatctgtgagttcttcttgcgaaaggggcatcccaaactcttggctcaagtcttttatcatagcagaggagggcagcaggtccctcaccgtcacgtcccagagggtggtgctgttatagcagatgtcgtggatcctggctagagcctggaagacccgcctccgctcagtgtctcgcaggaagaacaccgcctgctgcagcagcagctccgtgggctggaagaggtgcacgtggtacaggatggcctccaggtccccatagagccggctgcggaacagcagctgtgagttgtacagcaccttgtatttcctgtgttctgacctgggaatccagctttggtggttctcccacagctgcctcaagccttggtcggccaggccttccaggatgaaaaggtgtgtcttcccgtccagcaggtggaagccagtgagcacatccaggtgctgctgctcctggacccgcacacgcaccttgaaggctgacaggatctgctgcagggtcctgacagggtaggagtccaggccgagggccttagcgttgatcatggtgatgtcctgcagcaggctgtggagcagggagaccttcttaaagtcaaagacgaagatgatgcggccaaactgggagcccccaaggtcaggatcagcagctctggccccggccctcagtggcaccgcgatgtccactcgcaacttgagctgggagtcagcctctaggtagttgcccctgggcattgggccgtgctggtggccatctctggggaccccaagccccacaaccttccttctcctgctgtcctggccgcagtgtgtgggctgaacctcacagctgtggatggggacggccagattcaagtacttgtggccaaggaggaggtcagcaaaactgacctgggcgatgccataagggtaccacatcttgttctgggactcaaaggggttgttctctgtctctctgggagagatgagggcctggaagttgaggtatgaatccagagggtcctccccaaacagcacgggcttctgagaacactcctctgacttgcggtcccggtcgtgaacttccaccaccatgggggggccctccaggtattcccttaggtcactggggtgcagtgccccaaggaagatgacgttgatgtcctggaaataaacgtgggttccatggggctcccccttggtcttgtgaactggagtcttatggaactggtacttgcagtacacaggcatgcacagcctctctagttcctgaatgggtacaggctgtgatggaaggcaggaagcacacttgatctttatggtcaggggatttaaatcctgcttttgctcctcggtcatgatcggaacttctgtttttaaagtcaaaaggcaatctaaaatgttggcagacttctcactgccacgactcacgacagtttgccatccggcaaggagcggcatgacggccagctggatggagaaagcgctctgcttcctggggcctgtcagcgtggggtctgcctcttcttctgccaggggcttcttatgtctcctctggattttccttcttccctctgaatctttccctttaatttgagacctttgtctgtctaatatgtttgttaagctgctaagtgattcactctcaattaattccttgatctccatcatgcttgctcctgccaaagaaatggttggtgttcttgaaacactccattgaatcgtggaagaatcgtccattttgagggacttctcatattcctcactgttcttggaagaagtttcgggctctgcttggtgagaaccttgcaaagactttgggtgtttttctgttttttcttgttttcctggcggatgttcctggttcgactcttctctgacaatgttggtattctcaatgccctgttcagataattttctctgatttaaaaccaaatgtctcacttctgacttatgaaaagctcccacgtcgtctgtgaagccggcagtctttaatcggtaatatctgacttttcttgacatcttgtctttagtgttccagagcctcaaggtgattttgtggaaatttattttctttaataattcctttgtcacagtgatattaaaagtctgctcccacgacacccaggctttgtcaccttcgtgccacggcttcacagtctgcgagcggatgcgctgggcggcagcggggagttggaccgcgg

SEQ ID NO: 15603 - RNA, 6277 nt, Homo sapiens
  source 1..6277: mol_type = other RNA
gctgggattacaggcatgagccactgtgcccagccctggctgtattcttgaagctgcccggggaaggctcacgaagggaggagcatctggttgtacctgattctggagacagcattttacctgcccctttacccactgtactccatccaaaatgaccctgcagtgccctgcagaggtctcaggccttggcctagagaacagagggctttgctcgtgctccccgctctgtctgcagtgctcttcctcttctatagccactcgaccatatctaggaatgcccagctcagtctacctctgaccctcacagtcctgttgacctgaggttctggatcagtgtccccacaaagcccagtcgtgttgccaagtgatgggtgtaggcgccagcactgtggcacttgctgagagtggcatatgattttttgcaggtcctagccctgggggtagcccagacacccccccagtgctgacaggttatgtgctgtggagggtgctgaaatggtttctcctccagtgggctggaatcacagatgggctgtttacggagcaagtgccggctccaccccatgagatctgggggttagagatgagcaggatgagtcctttgtaactgagaatgaagctgtacccctttctctccctgcagccctgaatcacttgctgggggtctggaggaggggttcacccttagggctgcttcatggtgggtgggctgactttgtggaaaaatgcccccacttcagccatgtttgtcttatcacggtgcagaaagatcacccaccatctctccttttccttcccagatgctccagaaaacctagatgagcagattaagaaagtgtcccagcagatccttgagaagcgagcctatatctgtgcccaccctctggacaggacatgctgaggcaggggacagtgtcccctgctaccgcccgcccctacccatggcccgttgctggatgactgttactcttttttcagaaggtgttgggattatcacaggttaagccttttgttccccgtctgcacctgaagggttgtcgcctggcctgggagagcctcttccaggttttgacctgcaggcagtgctctctaacaggaccatcacagcttctgaactgagccggagagagagaatggaattgctgacccctggaactggcgggtattctggtcattgaggagacaccatagtggaaactggggcttatgctgctgcctccagggtgtgaggtgggtggggacctgtgtcaggtgtggatagccatttctgctcaaccacacattctctaagaaacagcttgaaagctctgtctgggtcattcatttaaactagaagcagaggcacttaaaacatgtaccaggaaccatttaacaaagaatataaaatgtcacaatctgtgtactgttagcctttgctgtacttgtcacactgttccttagaaccagcctttaatgggtgacagcaggaccctgagaaccaccctttggtgatggcctcgggtcccctttgtcctcaccctgcaaggagggcccagaatgctaaggagcagacacacagtgcaggccacaatcccttggggttatgagcccttagtttttatccttctcaggagatgatggggaggctgtctcagctgatgatgttcccacctagggactttagtttctttacaagaactggcttctactcttgaggagaggatgaatggtatctccaggccagcaggcctttgcatttctccagcctcccttctgctggcacttgaaagattacaccaggtcccagcgtgctcactgtggtgaactttaagctttgatgtggtccttgggtggtctggagctctaaaatgcctattgtggacactcccttgagcacagagaaggcagccgactctttttcctccaagtatattcccaatttactgtgatgctggaaataggcaaggaggagactgggaacttggagagctgagctggctgagtggggctggcctgagcattctgccaggggtttggtaactagtttttaaaatggggaaagtttgtaaatattgtgaccgtgtaaataacctctcagtgaaacctgaagttctgttagtgatagcagggcagcattttgcacaaaatgaagcatgcatacctctggacagaaggctgcttagagtttctttgcacaggagaagtttggggaggggctgtcagacccaccccccttctgtgcagccttctggaagggggcttcactctaggctggtggcgtgtaaggcctcagtcttacatgccaatggagaatggcaagttctccattcatccatctgggttgaaaaggcctagcgaccagttcaagcctctccctctcatctgtagttgctaacttttcttaaacatgttgtgggaagaggagaccccagcaagtgtttcttaagtgatttcaccagtgaaacccccaggagacttttgctgggaaggctggcagtggagctcactaggaagccttcttaccaaggaaaagccttgtgttcttaggctagacagctctcctagctggagcctccttgagagccacagcagtaactgtgggcctgggacatgcccacagagagcaggtctcttcaggcaacctgggagatctagggcctactggggagggagggagccaagtctaggcaaatggagaaagtgacatttcagcaaacttgttagcacttccatggagctgtgatcagttgtccttaggagtcgaggaggagaggaagccatcacgttcacctgacctagttttctgggagaagtttctctggcagaccttgtttttagataggctcatgtctctttctccctgaacaaaggttctggctctgttaaccaagtttgggttctatgttaacctccagatgatcctgagatcaattttcataaacagggataaagaggaagaggacttggagggactggtacagcaagacctacgtttcctgtctctgccttaccccaaagaaagaactgtcagtatctttgccgctggaaggtcccagtgaagcccagagcctctgcccccagctcttggctggacacctagagatcagtcatgggtaatagtgttgaagctcaggaagcctttagacctgtcttccaacttccccactttatagccaagaaaccagacccagggcatgaagggatttgcctcaagtcacacaaatgtcacacttggggctagaatcctggtctgagttccagcccagcattcaatctcttttttcagacccattctgcatcttgcttttcttagcatagaaagtttggttgatagtgtaaacaaaatggataccactgaagatgcagagtggcacagagctcctgcctgcccacggcatcaggaggcccagcttggcaaacccttgcctgttacctgttacaggctttggtgcgggcgaagggagcagctcgaggaaaggtggtggtttcttgtacagatcaaagtccacgtggtgcctgtcccagctccacctgtctcgatccaacacaggctccagtacattagcaaacagggagttttccttccactcctcattcagctctttgatgggtggcagcttgagatcctgaaagctgctttcggtgtcgctctgaagacctgtcacttggaatcccctggctgtgagccaggcctggcgggatttcttctgggctttcttctcctcttccttcaagtccaggggctccaccatggctgagaggtaatcctgtgagtacgtgaatctctttcttggctccttggctatctcttgatacagctccttcttggcaagctctgtagaattcatggtctgggtactatagttgtagacggccttgttggcaggggctgaaattttaatcaccttcgccacggacttcggaggcttcttgctgacctggtaggcttctgtgatatttttctggatgaaactgtgctttttgtctttgttcttcataagcatggcactccgccactgcaggtacttctcctggtgggcgtggatctctaaggtgagggtggagttccgactgtggtagtcctcaagattgggggcaggctgaggtggtagggcaaacagtttctcatctgtgagttcttcttgcgaaaggggcatcccaaactcttggctcaagtcttttatcatagcagaggagggcagcaggtccctcaccgtcacgtcccagagggtggtgctgttatagcagatgtcgtggatcctggctagagcctggaagacccgcctccgctcagtgtctcgcaggaagaacaccgcctgctgcagcagcagctccgtgggctggaagaggtgcacgtggtacaggatggcctccaggtccccatagagccggctgcggaacagcagctgtgagttgtacagcaccttgtatttcctgtgttctgacctgggaatccagctttggtggttctcccacagctgcctcaagccttggtcggccaggccttccaggatgaaaaggtgtgtcttcccgtccagcaggtggaagccagtgagcacatccaggtgctgctgctcctggacccgcacacgcaccttgaaggctgacaggatctgctgcagggtcctgacagggtaggagtccaggccgagggccttagcgttgatcatggtgatgtcctgcagcaggctgtggagcagggagaccttcttaaagtcaaagacgaagatgatgcggccaaactgggagcccccaaggtcaggatcagcagctctggccccggccctcagtggcaccgcgatgtccactcgcaacttgagctgggagtcagcctctaggtagttgcccctgggcattgggccgtgctggtggccatctctggggaccccaagccccacaaccttccttctcctgctgtcctggccgcagtgtgtgggctgaacctcacagctgtggatggggacggccagattcaagtacttgtggccaaggaggaggtcagcaaaactgacctgggcgatgccataagggtaccacatcttgttctgggactcaaaggggttgttctctgtctctctgggagagatgagggcctggaagttgaggtatgaatccagagggtcctccccaaacagcacgggcttctgagaacactcctctgacttgcggtcccggtcgtgaacttccaccaccatgggggggccctccaggtattcccttaggtcactggggtgcagtgccccaaggaagatgacgttgatgtcctggaaataaacgtgggttccatggggctcccccttggtcttgtgaactggagtcttatggaactggtacttgcagtacacaggcatgcacagcctctctagttcctgaatgggtacaggctgtgatggaaggcaggaagcacacttgatctttatggtcaggggatttaaatcctgcttttgctcctcggtcatgatcggaacttctgtttttaaagtcaaaaggcaatctaaaatgttggcagacttctcactgccacgactcacgacagtttgccatccggcaaggagcggcatgacggccagctggatggagaaagcgctctgcttcctggggcctgtcagcgtggggtctgcctcttcttctgccaggggcttcttatgtctcctctggattttccttcttccctctgaatctttccctttaatttgagacctttgtctgtctaatatgtttgttaagctgctaagtgattcactctcaattaattccttgatctccatcatgcttgctcctgccaaagaaatggttggtgttcttgaaacactccattgaatcgtggaagaatcgtccattttgagggacttctcatattcctcactgttcttggaagaagtttcgggctctgcttggtgagaaccttgcaaagactttgggtgtttttctgttttttcttgttttcctggcggatgttcctggttcgactcttctctgacaatgttggtattctcaatgccctgttcagataattttctctgatttaaaaccaaatgtctcacttctgacttatgaaaagctcccacgtcgtctgtgaagccggcagtctttaatcggtaatatctgacttttcttgacatcttgtctttagtgttccagagcctcaaggtgattttgtggaaatttattttctttaataattcctttgtcacagtgatattaaaagtctgctcccacgacacccaggctttgtcaccttcgtgccacggcttcacagtcttccgccagttccacgcgcgcctctgtggctacttcg

SEQ ID NO: 15604 - RNA, 12283 nt, Homo sapiens
  source 1..12283: mol_type = other RNA
gctgggattacaggcatgagccactgtgcccagccctggctgtattcttgaagctgcccggggaaggctcacgaagggaggagcatctggttgtacctgattctggagacagcattttacctgcccctttacccactgtactccatccaaaatgaccctgcagtgccctgcagaggtctcaggccttggcctagagaacagagggctttgctcgtgctccccgctctgtctgcagtgctcttcctcttctatagccactcgaccatatctaggaatgcccagctcagtctacctctgaccctcacagtcctgttgacctgaggttctggatcagtgtccccacaaagcccagtcgtgttgccaagtgatgggtgtaggcgccagcactgtggcacttgctgagagtggcatatgattttttgcaggtcctagccctgggggtagcccagacacccccccagtgctgacaggttatgtgctgtggagggtgctgaaatggtttctcctccagtgggctggaatcacagatgggctgtttacggagcaagtgccggctccaccccatgagatctgggggttagagatgagcaggatgagtcctttgtaactgagaatgaagctgtacccctttctctccctgcagccctgaatcacttgctgggggtctggaggaggggttcacccttagggctgcttcatggtgggtgggctgactttgtggaaaaatgcccccacttcagccatgtttgtcttatcacggtgcagaaagatcacccaccatctctccttttccttcccagatgctccagaaaacctagatgagcagattaagaaagtgtcccagcagatccttgagaagcgagcctatatctgtgcccaccctctggacaggacatgctgaggcaggggacagtgtcccctgctaccgcccgcccctacccatggcccgttgctggatgactgttactcttttttcagaaggtgttgggattatcacaggttaagccttttgttccccgtctgcacctgaagggttgtcgcctggcctgggagagcctcttccaggttttgacctgcaggcagtgctctctaacaggaccatcacagcttctgaactgagccggagagagagaatggaattgctgacccctggaactggcgggtattctggtcattgaggagacaccatagtggaaactggggcttatgctgctgcctccagggtgtgaggtgggtggggacctgtgtcaggtgtggatagccatttctgctcaaccacacattctctaagaaacagcttgaaagctctgtctgggtcattcatttaaactagaagcagaggcacttaaaacatgtaccaggaaccatttaacaaagaatataaaatgtcacaatctgtgtactgttagcctttgctgtacttgtcacactgttccttagaaccagcctttaatgggtgacagcaggaccctgagaaccaccctttggtgatggcctcgggtcccctttgtcctcaccctgcaaggagggcccagaatgctaaggagcagacacacagtgcaggccacaatcccttggggttatgagcccttagtttttatccttctcaggagatgatggggaggctgtctcagctgatgatgttcccacctagggactttagtttctttacaagaactggcttctactcttgaggagaggatgaatggtatctccaggccagcaggcctttgcatttctccagcctcccttctgctggcacttgaaagattacaccaggtcccagcgtgctcactgtggtgaactttaagctttgatgtggtccttgggtggtctggagctctaaaatgcctattgtggacactcccttgagcacagagaaggcagccgactctttttcctccaagtatattcccaatttactgtgatgctggaaataggcaaggaggagactgggaacttggagagctgagctggctgagtggggctggcctgagcattctgccaggggtttggtaactagtttttaaaatggggaaagtttgtaaatattgtgaccgtgtaaataacctctcagtgaaacctgaagttctgttagtgatagcagggcagcattttgcacaaaatgaagcatgcatacctctggacagaaggctgcttagagtttctttgcacaggagaagtttggggaggggctgtcagacccaccccccttctgtgcagccttctggaagggggcttcactctaggctggtggcgtgtaaggcctcagtcttacatgccaatggagaatggcaagttctccattcatccatctgggttgaaaaggcctagcgaccagttcaagcctctccctctcatctgtagttgctaacttttcttaaacatgttgtgggaagaggagaccccagcaagtgtttcttaagtgatttcaccagtgaaacccccaggagacttttgctgggaaggctggcagtggagctcactaggaagccttcttaccaaggaaaagccttgtgttcttaggctagacagctctcctagctggagcctccttgagagccacagcagtaactgtgggcctgggacatgcccacagagagcaggtctcttcaggcaacctgggagatctagggcctactggggagggagggagccaagtctaggcaaatggagaaagtgacatttcagcaaacttgttagcacttccatggagctgtgatcagttgtccttaggagtcgaggaggagaggaagccatcacgttcacctgacctagttttctgggagaagtttctctggcagaccttgtttttagataggctcatgtctctttctccctgaacaaaggttctggctctgttaaccaagtttgggttctatgttaacctccagatgatcctgagatcaattttcataaacagggataaagaggaagaggacttggagggactggtacagcaagacctacgtttcctgtctctgccttaccccaaagaaagaactgtcagtatctttgccgctggaaggtcccagtgaagcccagagcctctgcccccagctcttggctggacacctagagatcagtcatgggtaatagtgttgaagctcaggaagcctttagacctgtcttccaacttccccactttatagccaagaaaccagacccagggcatgaagggatttgcctcaagtcacacaaatgtcacacttggggctagaatcctggtctgagttccagcccagcattcaatctcttttttcagacccattctgcatcttgcttttcttagcatagaaagtttggttgatagtgtaaacaaaatggataccactgaagatgcagagtggcacagagctcctgcctgcccacggcatcaggaggcccagcttggcaaacccttgcctgttacctgttacaggctttggtgcgggcgaagggagcagctcgaggaaaggtggtggtttcttgtacagatcaaagtccacgtggtgcctgtcccagctccacctgtctcgatccaacacaggctccagtacattagcaaacagggagttttccttccactcctcattcagctctttgatgggtggcagcttgagatcctgaaagctgctttcggtgtcgctctgaagacctgtcacttggaatcccctggctgtgagccaggcctggcgggatttcttctgggctttcttctcctcttccttcaagtccaggggctccaccatggctgagaggtaatcctgtgagtacgtgaatctctttcttggctccttggctatctcttgatacagctccttcttggcaagctctgtagaattcatggtctgggtactatagttgtagacggccttgttggcaggggctgaaattttaatcaccttcgccacggacttcggaggcttcttgctgacctggtaggcttctgtgatatttttctggatgaaactgtgctttttgtctttgttcttcataagcatggcactccgccactgcaggtacttctcctggtgggcgtggatctctaaggtgagggtggagttccgactgtggtagtcctcaagattgggggcaggctgaggtggtagggcaaacagtttctcatctgtgagttcttcttgcgaaaggggcatcccaaactcttggctcaagtcttttatcatagcagaggagggcagcaggtccctcaccgtcacgtcccagagggtggtgctgttatagcagatgtcgtggatcctggctagagcctggaagacccgcctccgctcagtgtctcgcaggaagaacaccgcctgctgcagcagcagctccgtgggctggaagaggtgcacgtggtacaggatggcctccaggtccccatagagccggctgcggaacagcagctgtgagttgtacagcaccttgtatttcctgtgttctgacctgggaatccagctttggtggttctcccacagctgcctcaagccttggtcggccaggccttccaggatgaaaaggtgtgtcttcccgtccagcaggtggaagccagtgagcacatccaggtgctgctgctcctggacccgcacacgcaccttgaaggctgacaggatctgctgcagggtcctgacagggtaggagtccaggccgagggccttagcgttgatcatggtgatgtcctgcagcaggctgtggagcagggagaccttcttaaagtcaaagacgaagatgatgcggccaaactgggagcccccaaggtcaggatcagcagctctggccccggccctcagtggcaccgcgatgtccactcgcaacttgagctgggagtcagcctctaggtagttgcccctgggcattgggccgtgctggtggccatctctggggaccccaagccccacaaccttccttctcctgctgtcctggccgcagtgtgtgggctgaacctcacagctgtggatggggacggccagattcaagtacttgtggccaaggaggaggtcagcaaaactgacctgggcgatgccataagggtaccacatcttgttctgggactcaaaggggttgttctctgtctctctgggagagatgagggcctggaagttgaggtatgaatccagagggtcctccccaaacagcacgggcttctgagaacactcctctgacttgcggtcccggtcgtgaacttccaccaccatgggggggccctccaggtattcccttaggtcactggggtgcagtgccccaaggaagatgacgttgatgtcctggaaataaacgtgggttccatggggctcccccttggtcttgtgaactggagtcttatggaactggtacttgcagtacacaggcatgcacagcctctctagttcctgaatgggtacaggctgtgatggaaggcaggaagcacacttgatctttatggtcaggggatttaaatcctgcttttgctcctcggtcatgatcggaacttctgtttttaaagtcaaaaggcaatctaaaatgttggcagacttctcactgccacgactcacgacagtttgccatccggcaaggagcggcatgacggccagctggatggagaaagcgctctgcttcctggggcctgtcagcgtggggtctgcctcttcttctgccaggggcttcttatgtctcctctggattttccttcttccctctgaatctttccctttaatttgagacctttgtctgtctaatatgtttgttaagctgctaagtgattcactctcaattaattccttgatctccatcatgcttgctcctgccaaagaaatggttggtgttcttgaaacactccattgaatcgtggaagaatcgtccattttgagggacttctcatattcctcactgttcttggaagaagtttcgggctctgcttggtgagaaccttgcaaagactttgggtgtttttctgttttttcttgttttcctggcggatgttcctggttcgactcttctctgacaatgttggtattctcaatgccctgttcagataattttctctgatttaaaaccaaatgtctcacttctgacttatgaaaagctcccacgtcgtctgtgaagccggcagtctttaatcggtaatatctgacttttcttgacatcttgtctttagtgttccagagcctcaaggtgattttgtggaaatttattttctttaataattcctttgtcacagtgatattaaaagtctgctcccacgacacccaggctttgtcaccttcgtgccacggcttcacagtctttactcctgactccaggaatactttggccaccattggaaatagcaatatgtcaacttttttaggttcttcatcgtccggcagaaggaaatactcaatgtggtaaaaacgacgcatctttgtaacagaactgtctgttttagggtgtttcttatatttttcaatcaaacttgcatattttcccttccatattcacagggaaggccagtgagatggtgaatttgcaggggaccacgtggggcacgtcggagctgaaagtgctggcaggctcagatgaggactcgatgctgctgcacgggcggtcagagtcagactcctgggccctggccttggccttcaggtgttcctccacgtcacactcgctcgtggactggtaaaagctagtgatggaggagatgggctctatgcttgcggggtcctcttcccactcccaggcatgtagcgacatgctgcagagcgcactgctggccgccggcgctcctgcgagcggatgcgctgggcggcagcggggagttggaccgcggcggcaactcccgtaccggatccacagccacctgggcgaagagactccaagactgagaggagcgtccgccggtgcagggagggccgcaggcccagccactcagctacgtttggcggttgctaggagacgcgagggcgtgcggcctgggggcggggctccgcggggcggggctttccccctcagccactgcgcgcagtttgtcaaatggctacatccaggttcagaaaccagctgccttcattccttcactcatgcattcactcattaaggagtttctactcggaacgtcagcacctactataagcctggtccttgcccgtacgatgggaggtaggggttgatggctccttcctccccctccatcagctcccacctcccattctttaataaaagcaaaggaagctgtgggctctgcaaactccagacctccccacgatccctctcattagattctctgcttctgtcgccgatgtccttaaaaaccagacctccccacgatccctctcattagattctctgcttctgtcgctgatgtccttaaaatagcatgagaattcttgttagtgatcatgagcgccaactcagagatcagaaaacaaagcttagagaggtgaagcgattcgcccgaggtcacacagcaagtagggcgcagcactgtgttgaaatccggactgcctgactccaaagcctccgctcgtctgctaaaccacccaagctgagagccctggctgcggctcctaatgtagaggacctcagcacagcaagcggctgggacagagggctggggtaggcctcatggaggaagtgagcaacgccaaatctggggggtgactaggcagaggcggtgaaagcaagagaaagcatcccaggtagaggaacagcatatgcaaaggcccatagaggtgaaagggcatggcaagtttcaggaatgggtggcgaggctgtagcagtgtgcagggcccatggtacatagccccacagggcaggttagggcacaggactatgggcaatggggagccaaggcaggtcttctgttgagggagggcaccctgctccggcagtcagtttgttcaagagaatgggagctgaggctacacacaagcttggctattaagaaaactttagctgagttgagctatgacctactttgtgtcaaagagcaaaactgtggcgcagctggggctgagacccaagtcctgagcctcccagtgcatgcctccccagaccgctctcagggcatgggacagcccctttaatactgggtgctccaatactcctcgggttcagtctgaaaaacagcctcaagtacagctgttagggaagacaccaaatggcagtgggccctgtgaggagtgggttcaaactcttagcacgagaacggcaaccaccttgcccacaccccacctgcagcagcctggagactgctgtctgtatgccaggaagtgctcaggagacacatgaagggctggaagaatacaaagctactcagatacaccagcccccaaaagggccctttaacaagggcagttcaacactaccaccactcttggacagacatcaggcctcctgctccccaggtcctacccactggcctgaggctggtttccctccaaaggttcctagatcacatcaccacctaggacagaagccaatctcttcccaagctcaatagtgagaggccagaggtcttggaccaagggccaatgtgccatcctggatgtgcactggaaacacctacatgtcaaaaatacaattctgaggcttcattaaagacctgtggaagtgactctccaggggtggagcttagaaaccagtggcagattgtattttccaaagacagccacctcaaaagatcccctcccacataatcttccggcaggcattgtgaggttcacattcctcccacccagttggggggtctagtctccttctctggaaactgggcagacctctgtgactggctcagtcaaaagagtgcagaggaaatgacactatgtgatttctgaggccaggtcatataaattccatctacctctgccctgttcttttgaggtatagtattcatgctaggaatccagctagcatgttgtgaggaagcccaagcagccatgtgaaatggccacatgaaactgttgtgactgacggttcccagccaattgcagcctcaacccccagacatatgagagtgcaagacttcaaatgatcccagccctcagtctttgagccaccctggctgacattgaggaacagaaacaagctgtctccatcatgagaaattgtagatttataagcaaattgttgctctcttaaaccactaagttttggggtgatttgttgtgcaataaataataggaacgggagccatatttttaaattaccaccaagattgtattgcacaaccagaatatggaaccactgccctgagagagatggtgtctgggtcaagacctagggcatcacaggatgaagtgagggcaaaggtgtgctacccactactcaggtatgagacagtggtgggtctacaaccctacctcagtgaagatggcttcagggctggcagatcagaagcaaaggaaggggggcttctgtttcagttatctgttactgagtaaaaaccatccccaaacttaatggtgtcaaacaaacacttgttatttctcaccactccatgcatcagctgagtagttctctgctggcctcgcctgggctcactccctatgctgtgctcagctggaggaccaacatggctggaagctgccagaagtcctcacttgcatgtctggcagttgctgctggctcttcgtgggcccgctggttcccctccatgggttcccccgcccccagtggtacaccagcttccttctatgtggtgcctcatctcctcatagcccggcctggcttcctcagatggcattctcagagcagggatcccagagggcaaagaagaagttgcaaggcctcttgggacctaggcgtggaaccagcaccatgtcactctgctacatgccattaaccaaagcaagtcatgaggctggccccacttcaaggggatgaagacatggactgtacatctggtaagcagagggacaagcatccaggggcaggaggtgttcaaggtcactgaacaatccatcccttcatccttactctgccgggtggagggttcccaagctcccacaggctatgtagaggccttcctgaagctatcccaagactctggcagctggaagcatattgggaatcagctacatacaccttcttcttgccccttccccatttttaacagctttattgaagtattttttatttaataaaatccatccatttcaagcgtagaattcaatgattttcagtaactttacctagtgctgtaatcatcatcataaattcattttagaacattttcatccccctaataagacttcatgcacatttataattaatctctgttccaactcccagtcctaggcaaccatatctactttgtttctaaaaattggccttttctagacatttcctataaattgagtcagacactgtgttctggctttgtgactggtttctttcacctaccgttatgtttccaaggtttatttatgttgaggcatgtgtcagtatttcattccttttcatgactgaataatattctattgtatggacagaccacagtttgcctatccattcatcagttaatgggcatttggcttgggcatttagacatttatgaacaacgttgctatgaacattcccacacaagtctttgtgtggatgtgttttcatctctcttgggtcgatatctaggagtggaagagttgggtcgtatggtcattttgtgattaacttcttgagaaactgccaaactatcttccacaggggctgcatcattttgtgttcccatcaacaacatgaagtttcctgtttctccaaattcttgacaagatttattgcctgttttattcactacagctattctcatgagtataatatagtatttcatcatagttttcatgtgcatttccctaacaagaatactgagattgttttatgcacatgttggctatttatacaacttctttggtgaaatgtctgtttgtatcttcacccactttttgattggattgtttgtcttcttgttactgagttgttaagagttcattgtaaattcggaatataagtcctttactgggcatatgttttacaaatattttctcctagtctcttgttcgtcatattttcttaatagtgtcttttgaagtgcaaatgttttgaactttgatgaaggtccgattcatcatttttttcttttttggatcatgcatttggtgtcgtatctaagaaatctttgactaacaacaggcctatttttaatagaagtaaagcttggtgtctgaacactaagcaaatctactaaccaagacccctaaaaacccaaaagctttatgacactgaaaataatggcccaaggacattcccagacagttctgggctctggatagaacaacacaagtttccaaaaaacaggctgataataccacaagcttataaaatatgtatactccttggcccagtaataaatcactcaagatatggcacaaactgttcacagtatggtttttgcggagaaaagctgaaaaccacctcagtgggcatctgtgggggatgacaaagcaccttatagttcatccccagggagcacagagcagcctctggagcagtgtctgcaaagaaaccacagccaagctgtttacaaagctcagttcctgtgcaaagaaagatcccaatggcgccctttccactgtgcttttcatgtcaagttgaatgagctacgatttgcacactgtaaaattcagatgtacacagtcatgcaaccactacaccatgaagatagagtatttcaatcactccaaaaagttctttcatgcccaaatacatagaaaagtctggaaataaatacatcagaaatacacagtgatcctctcttggtggcagaatggtggatgatttttgctttttagcattttcccggacctttaaaagacactttaaacaatatactatttgaaatggctcaaacaatactgaactgacttcagaaaatcatttctttgccacagccctgactctctcccacacagacacacgcccatccccccagctcatacaaaagaacgcaaggagacctctgagtttgctcactttgaaccttaaacaaaaaccttgtggatgcaaccagaattatttcagaggtgcctggtaacaccgcagggcagacagacaggcctgacagcaaaccattatcaacccttacttccctgagctgtaggggagtggaggccggcaacggctcccagcaagacatttaaaagctttcttttcaatattgactggcccaggaaagctactgttcaaaggattccttcaccagctgcagggatggggggtggggagggtgttgcactcttgcctgggctaccagctcttagggctgacatgaaataaaatcaggttctttttttttttt

SEQ ID NO: 15605 - RNA, 6888 nt, Homo sapiens
  source 1..6888: mol_type = other RNA
gctgggattacaggcatgagccactgtgcccagccctggctgtattcttgaagctgcccggggaaggctcacgaagggaggagcatctggttgtacctgattctggagacagcattttacctgcccctttacccactgtactccatccaaaatgaccctgcagtgccctgcagaggtctcaggccttggcctagagaacagagggctttgctcgtgctccccgctctgtctgcagtgctcttcctcttctatagccactcgaccatatctaggaatgcccagctcagtctacctctgaccctcacagtcctgttgacctgaggttctggatcagtgtccccacaaagcccagtcgtgttgccaagtgatgggtgtaggcgccagcactgtggcacttgctgagagtggcatatgattttttgcaggtcctagccctgggggtagcccagacacccccccagtgctgacaggttatgtgctgtggagggtgctgaaatggtttctcctccagtgggctggaatcacagatgggctgtttacggagcaagtgccggctccaccccatgagatctgggggttagagatgagcaggatgagtcctttgtaactgagaatgaagctgtacccctttctctccctgcagccctgaatcacttgctgggggtctggaggaggggttcacccttagggctgcttcatggtgggtgggctgactttgtggaaaaatgcccccacttcagccatgtttgtcttatcacggtgcagaaagatcacccaccatctctccttttccttcccagatgctccagaaaacctagatgagcagattaagaaagtgtcccagcagatccttgagaagcgagcctatatctgtgcccaccctctggacaggacatgctgaggcaggggacagtgtcccctgctaccgcccgcccctacccatggcccgttgctggatgactgttactcttttttcagaaggtgttgggattatcacaggttaagccttttgttccccgtctgcacctgaagggttgtcgcctggcctgggagagcctcttccaggttttgacctgcaggcagtgctctctaacaggaccatcacagcttctgaactgagccggagagagagaatggaattgctgacccctggaactggcgggtattctggtcattgaggagacaccatagtggaaactggggcttatgctgctgcctccagggtgtgaggtgggtggggacctgtgtcaggtgtggatagccatttctgctcaaccacacattctctaagaaacagcttgaaagctctgtctgggtcattcatttaaactagaagcagaggcacttaaaacatgtaccaggaaccatttaacaaagaatataaaatgtcacaatctgtgtactgttagcctttgctgtacttgtcacactgttccttagaaccagcctttaatgggtgacagcaggaccctgagaaccaccctttggtgatggcctcgggtcccctttgtcctcaccctgcaaggagggcccagaatgctaaggagcagacacacagtgcaggccacaatcccttggggttatgagcccttagtttttatccttctcaggagatgatggggaggctgtctcagctgatgatgttcccacctagggactttagtttctttacaagaactggcttctactcttgaggagaggatgaatggtatctccaggccagcaggcctttgcatttctccagcctcccttctgctggcacttgaaagattacaccaggtcccagcgtgctcactgtggtgaactttaagctttgatgtggtccttgggtggtctggagctctaaaatgcctattgtggacactcccttgagcacagagaaggcagccgactctttttcctccaagtatattcccaatttactgtgatgctggaaataggcaaggaggagactgggaacttggagagctgagctggctgagtggggctggcctgagcattctgccaggggtttggtaactagtttttaaaatggggaaagtttgtaaatattgtgaccgtgtaaataacctctcagtgaaacctgaagttctgttagtgatagcagggcagcattttgcacaaaatgaagcatgcatacctctggacagaaggctgcttagagtttctttgcacaggagaagtttggggaggggctgtcagacccaccccccttctgtgcagccttctggaagggggcttcactctaggctggtggcgtgtaaggcctcagtcttacatgccaatggagaatggcaagttctccattcatccatctgggttgaaaaggcctagcgaccagttcaagcctctccctctcatctgtagttgctaacttttcttaaacatgttgtgggaagaggagaccccagcaagtgtttcttaagtgatttcaccagtgaaacccccaggagacttttgctgggaaggctggcagtggagctcactaggaagccttcttaccaaggaaaagccttgtgttcttaggctagacagctctcctagctggagcctccttgagagccacagcagtaactgtgggcctgggacatgcccacagagagcaggtctcttcaggcaacctgggagatctagggcctactggggagggagggagccaagtctaggcaaatggagaaagtgacatttcagcaaacttgttagcacttccatggagctgtgatcagttgtccttaggagtcgaggaggagaggaagccatcacgttcacctgacctagttttctgggagaagtttctctggcagaccttgtttttagataggctcatgtctctttctccctgaacaaaggttctggctctgttaaccaagtttgggttctatgttaacctccagatgatcctgagatcaattttcataaacagggataaagaggaagaggacttggagggactggtacagcaagacctacgtttcctgtctctgccttaccccaaagaaagaactgtcagtatctttgccgctggaaggtcccagtgaagcccagagcctctgcccccagctcttggctggacacctagagatcagtcatgggtaatagtgttgaagctcaggaagcctttagacctgtcttccaacttccccactttatagccaagaaaccagacccagggcatgaagggatttgcctcaagtcacacaaatgtcacacttggggctagaatcctggtctgagttccagcccagcattcaatctcttttttcagacccattctgcatcttgcttttcttagcatagaaagtttggttgatagtgtaaacaaaatggataccactgaagatgcagagtggcacagagctcctgcctgcccacggcatcaggaggcccagcttggcaaacccttgcctgttacctgttacaggctttggtgcgggcgaagggagcagctcgaggaaaggtggtggtttcttgtacagatcaaagtccacgtggtgcctgtcccagctccacctgtctcgatccaacacaggctccagtacattagcaaacagggagttttccttccactcctcattcagctctttgatgggtggcagcttgagatcctgaaagctgctttcggtgtcgctctgaagacctgtcacttggaatcccctggctgtgagccaggcctggcgggatttcttctgggctttcttctcctcttccttcaagtccaggggctccaccatggctgagaggtaatcctgtgagtacgtgaatctctttcttggctccttggctatctcttgatacagctccttcttggcaagctctgtagaattcatggtctgggtactatagttgtagacggccttgttggcaggggctgaaattttaatcaccttcgccacggacttcggaggcttcttgctgacctggtaggcttctgtgatatttttctggatgaaactgtgctttttgtctttgttcttcataagcatggcactccgccactgcaggtacttctcctggtgggcgtggatctctaaggtgagggtggagttccgactgtggtagtcctcaagattgggggcaggctgaggtggtagggcaaacagtttctcatctgtgagttcttcttgcgaaaggggcatcccaaactcttggctcaagtcttttatcatagcagaggagggcagcaggtccctcaccgtcacgtcccagagggtggtgctgttatagcagatgtcgtggatcctggctagagcctggaagacccgcctccgctcagtgtctcgcaggaagaacaccgcctgctgcagcagcagctccgtgggctggaagaggtgcacgtggtacaggatggcctccaggtccccatagagccggctgcggaacagcagctgtgagttgtacagcaccttgtatttcctgtgttctgacctgggaatccagctttggtggttctcccacagctgcctcaagccttggtcggccaggccttccaggatgaaaaggtgtgtcttcccgtccagcaggtggaagccagtgagcacatccaggtgctgctgctcctggacccgcacacgcaccttgaaggctgacaggatctgctgcagggtcctgacagggtaggagtccaggccgagggccttagcgttgatcatggtgatgtcctgcagcaggctgtggagcagggagaccttcttaaagtcaaagacgaagatgatgcggccaaactgggagcccccaaggtcaggatcagcagctctggccccggccctcagtggcaccgcgatgtccactcgcaacttgagctgggagtcagcctctaggtagttgcccctgggcattgggccgtgctggtggccatctctggggaccccaagccccacaaccttccttctcctgctgtcctggccgcagtgtgtgggctgaacctcacagctgtggatggggacggccagattcaagtacttgtggccaaggaggaggtcagcaaaactgacctgggcgatgccataagggtaccacatcttgttctgggactcaaaggggttgttctctgtctctctgggagagatgagggcctggaagttgaggtatgaatccagagggtcctccccaaacagcacgggcttctgagaacactcctctgacttgcggtcccggtcgtgaacttccaccaccatgggggggccctccaggtattcccttaggtcactggggtgcagtgccccaaggaagatgacgttgatgtcctggaaataaacgtgggttccatggggctcccccttggtcttgtgaactggagtcttatggaactggtacttgcagtacacaggcatgcacagcctctctagttcctgaatgggtacaggctgtgatggaaggcaggaagcacacttgatctttatggtcaggggatttaaatcctgcttttgctcctcggtcatgatcggaacttctgtttttaaagtcaaaaggcaatctaaaatgttggcagacttctcactgccacgactcacgacagtttgccatccggcaaggagcggcatgacggccagctggatggagaaagcgctctgcttcctggggcctgtcagcgtggggtctgcctcttcttctgccaggggcttcttatgtctcctctggattttccttcttccctctgaatctttccctttaatttgagacctttgtctgtctaatatgtttgttaagctgctaagtgattcactctcaattaattccttgatctccatcatgcttgctcctgccaaagaaatggttggtgttcttgaaacactccattgaatcgtggaagaatcgtccattttgagggacttctcatattcctcactgttcttggaagaagtttcgggctctgcttggtgagaaccttgcaaagactttgggtgtttttctgttttttcttgttttcctggcggatgttcctggttcgactcttctctgacaatgttggtattctcaatgccctgttcagataattttctctgatttaaaaccaaatgtctcacttctgacttatgaaaagctcccacgtcgtctgtgaagccggcagtctttaatcggtaatatctgacttttcttgacatcttgtctttagtgttccagagcctcaaggtgattttgtggaaatttattttctttaataattcctttgtcacagtgatattaaaagtctgctcccacgacacccaggctttgtcaccttcgtgccacggcttcacagtctttactcctgactccaggaatactttggccaccattggaaatagcaatatgtcaacttttttaggttcttcatcgtccggcagaaggaaatactcaatgtggtaaaaacgacgcatctttgtaacagaactgtctgttttagggtgtttcttatatttttcaatcaaacttgcatattttcccttctgacccatattcacagggaaggccagtgagatggtgaatttgcaggggaccacgtggggcacgtcggagctgaaagtgctggcaggctcagatgaggactcgatgctgctgcacgggcggtcagagtcagactcctgggccctggccttggccttcaggtgttcctccacgtcacactcgctcgtggactggtaaaagctagtgatggaggagatgggctctatgcttgcggggtcctcttcccactcccaggcatgtagcgacatgctgcagagcgcactgctggccgccggcgctcctgcgagcggatgcgctgggcggcagcggggagttggaccgcggcggcaactcccgtaccggatccacagccacctgggcgaagagactccaagactgagaggagcgtccgccggtgcagggagggccgcaggcccagccactcagctacgtttggcggttgct

SEQ ID NO: 15606 - RNA, 7338 nt, Homo sapiens
  source 1..7338: mol_type = other RNA
gctgggattacaggcatgagccactgtgcccagccctggctgtattcttgaagctgcccggggaaggctcacgaagggaggagcatctggttgtacctgattctggagacagcattttacctgcccctttacccactgtactccatccaaaatgaccctgcagtgccctgcagaggtctcaggccttggcctagagaacagagggctttgctcgtgctccccgctctgtctgcagtgctcttcctcttctatagccactcgaccatatctaggaatgcccagctcagtctacctctgaccctcacagtcctgttgacctgaggttctggatcagtgtccccacaaagcccagtcgtgttgccaagtgatgggtgtaggcgccagcactgtggcacttgctgagagtggcatatgattttttgcaggtcctagccctgggggtagcccagacacccccccagtgctgacaggttatgtgctgtggagggtgctgaaatggtttctcctccagtgggctggaatcacagatgggctgtttacggagcaagtgccggctccaccccatgagatctgggggttagagatgagcaggatgagtcctttgtaactgagaatgaagctgtacccctttctctccctgcagccctgaatcacttgctgggggtctggaggaggggttcacccttagggctgcttcatggtgggtgggctgactttgtggaaaaatgcccccacttcagccatgtttgtcttatcacggtgcagaaagatcacccaccatctctccttttccttcccagatgctccagaaaacctagatgagcagattaagaaagtgtcccagcagatccttgagaagcgagcctatatctgtgcccaccctctggacaggacatgctgaggcaggggacagtgtcccctgctaccgcccgcccctacccatggcccgttgctggatgactgttactcttttttcagaaggtgttgggattatcacaggttaagccttttgttccccgtctgcacctgaagggttgtcgcctggcctgggagagcctcttccaggttttgacctgcaggcagtgctctctaacaggaccatcacagcttctgaactgagccggagagagagaatggaattgctgacccctggaactggcgggtattctggtcattgaggagacaccatagtggaaactggggcttatgctgctgcctccagggtgtgaggtgggtggggacctgtgtcaggtgtggatagccatttctgctcaaccacacattctctaagaaacagcttgaaagctctgtctgggtcattcatttaaactagaagcagaggcacttaaaacatgtaccaggaaccatttaacaaagaatataaaatgtcacaatctgtgtactgttagcctttgctgtacttgtcacactgttccttagaaccagcctttaatgggtgacagcaggaccctgagaaccaccctttggtgatggcctcgggtcccctttgtcctcaccctgcaaggagggcccagaatgctaaggagcagacacacagtgcaggccacaatcccttggggttatgagcccttagtttttatccttctcaggagatgatggggaggctgtctcagctgatgatgttcccacctagggactttagtttctttacaagaactggcttctactcttgaggagaggatgaatggtatctccaggccagcaggcctttgcatttctccagcctcccttctgctggcacttgaaagattacaccaggtcccagcgtgctcactgtggtgaactttaagctttgatgtggtccttgggtggtctggagctctaaaatgcctattgtggacactcccttgagcacagagaaggcagccgactctttttcctccaagtatattcccaatttactgtgatgctggaaataggcaaggaggagactgggaacttggagagctgagctggctgagtggggctggcctgagcattctgccaggggtttggtaactagtttttaaaatggggaaagtttgtaaatattgtgaccgtgtaaataacctctcagtgaaacctgaagttctgttagtgatagcagggcagcattttgcacaaaatgaagcatgcatacctctggacagaaggctgcttagagtttctttgcacaggagaagtttggggaggggctgtcagacccaccccccttctgtgcagccttctggaagggggcttcactctaggctggtggcgtgtaaggcctcagtcttacatgccaatggagaatggcaagttctccattcatccatctgggttgaaaaggcctagcgaccagttcaagcctctccctctcatctgtagttgctaacttttcttaaacatgttgtgggaagaggagaccccagcaagtgtttcttaagtgatttcaccagtgaaacccccaggagacttttgctgggaaggctggcagtggagctcactaggaagccttcttaccaaggaaaagccttgtgttcttaggctagacagctctcctagctggagcctccttgagagccacagcagtaactgtgggcctgggacatgcccacagagagcaggtctcttcaggcaacctgggagatctagggcctactggggagggagggagccaagtctaggcaaatggagaaagtgacatttcagcaaacttgttagcacttccatggagctgtgatcagttgtccttaggagtcgaggaggagaggaagccatcacgttcacctgacctagttttctgggagaagtttctctggcagaccttgtttttagataggctcatgtctctttctccctgaacaaaggttctggctctgttaaccaagtttgggttctatgttaacctccagatgatcctgagatcaattttcataaacagggataaagaggaagaggacttggagggactggtacagcaagacctacgtttcctgtctctgccttaccccaaagaaagaactgtcagtatctttgccgctggaaggtcccagtgaagcccagagcctctgcccccagctcttggctggacacctagagatcagtcatgggtaatagtgttgaagctcaggaagcctttagacctgtcttccaacttccccactttatagccaagaaaccagacccagggcatgaagggatttgcctcaagtcacacaaatgtcacacttggggctagaatcctggtctgagttccagcccagcattcaatctcttttttcagacccattctgcatcttgcttttcttagcatagaaagtttggttgatagtgtaaacaaaatggataccactgaagatgcagagtggcacagagctcctgcctgcccacggcatcaggaggcccagcttggcaaacccttgcctgttacctgttacaggctttggtgcgggcgaagggagcagctcgaggaaaggtggtggtttcttgtacagatcaaagtccacgtggtgcctgtcccagctccacctgtctcgatccaacacaggctccagtacattagcaaacagggagttttccttccactcctcattcagctctttgatgggtggcagcttgagatcctgaaagctgctttcggtgtcgctctgaagacctgtcacttggaatcccctggctgtgagccaggcctggcgggatttcttctgggctttcttctcctcttccttcaagtccaggggctccaccatggctgagaggtaatcctgtgagtacgtgaatctctttcttggctccttggctatctcttgatacagctccttcttggcaagctctgtagaattcatggtctgggtactatagttgtagacggccttgttggcaggggctgaaattttaatcaccttcgccacggacttcggaggcttcttgctgacctggtaggcttctgtgatatttttctggatgaaactgtgctttttgtctttgttcttcataagcatggcactccgccactgcaggtacttctcctggtgggcgtggatctctaaggtgagggtggagttccgactgtggtagtcctcaagattgggggcaggctgaggtggtagggcaaacagtttctcatctgtgagttcttcttgcgaaaggggcatcccaaactcttggctcaagtcttttatcatagcagaggagggcagcaggtccctcaccgtcacgtcccagagggtggtgctgttatagcagatgtcgtggatcctggctagagcctggaagacccgcctccgctcagtgtctcgcaggaagaacaccgcctgctgcagcagcagctccgtgggctggaagaggtgcacgtggtacaggatggcctccaggtccccatagagccggctgcggaacagcagctgtgagttgtacagcaccttgtatttcctgtgttctgacctgggaatccagctttggtggttctcccacagctgcctcaagccttggtcggccaggccttccaggatgaaaaggtgtgtcttcccgtccagcaggtggaagccagtgagcacatccaggtgctgctgctcctggacccgcacacgcaccttgaaggctgacaggatctgctgcagggtcctgacagggtaggagtccaggccgagggccttagcgttgatcatggtgatgtcctgcagcaggctgtggagcagggagaccttcttaaagtcaaagacgaagatgatgcggccaaactgggagcccccaaggtcaggatcagcagctctggccccggccctcagtggcaccgcgatgtccactcgcaacttgagctgggagtcagcctctaggtagttgcccctgggcattgggccgtgctggtggccatctctggggaccccaagccccacaaccttccttctcctgctgtcctggccgcagtgtgtgggctgaacctcacagctgtggatggggacggccagattcaagtacttgtggccaaggaggaggtcagcaaaactgacctgggcgatgccataagggtaccacatcttgttctgggactcaaaggggttgttctctgtctctctgggagagatgagggcctggaagttgaggtatgaatccagagggtcctccccaaacagcacgggcttctgagaacactcctctgacttgcggtcccggtcgtgaacttccaccaccatgggggggccctccaggtattcccttaggtcactggggtgcagtgccccaaggaagatgacgttgatgtcctggaaataaacgtgggttccatggggctcccccttggtcttgtgaactggagtcttatggaactggtacttgcagtacacaggcatgcacagcctctctagttcctgaatgggtacaggctgtgatggaaggcaggaagcacacttgatctttatggtcaggggatttaaatcctgcttttgctcctcggtcatgatcggaacttctgtttttaaagtcaaaaggcaatctaaaatgttggcagacttctcactgccacgactcacgacagtttgccatccggcaaggagcggcatgacggccagctggatggagaaagcgctctgcttcctggggcctgtcagcgtggggtctgcctcttcttctgccaggggcttcttatgtctcctctggattttccttcttccctctgaatctttccctttaatttgagacctttgtctgtctaatatgtttgttaagctgctaagtgattcactctcaattaattccttgatctccatcatgcttgctcctgccaaagaaatggttggtgttcttgaaacactccattgaatcgtggaagaatcgtccattttgagggacttctcatattcctcactgttcttggaagaagtttcgggctctgcttggtgagaaccttgcaaagactttgggtgtttttctgttttttcttgttttcctggcggatgttcctggttcgactcttctctgacaatgttggtattctcaatgccctgttcagataattttctctgatttaaaaccaaatgtctcacttctgacttatgaaaagctcccacgtcgtctgtgaagccggcagtctttaatcggtaatatctgacttttcttgacatcttgtctttagtgttccagagcctcaaggtgattttgtggaaatttattttctttaataattcctttgtcacagtgatattaaaagtctgctcccacgacacccaggctttgtcaccttcgtgccacggcttcacagtctttactcctgactccaggaatactttggccaccattggaaatagcaatatgtcaacttttttaggttcttcatcgtccggcagaaggaaatactcaatgtggtaaaaacgacgcatctttgtaacagaactgtctgttttagggtgtttcttatatttttcaatcaaacttgcatattttcccttctgacccatattcacagggaaggccagtgagatggtgaatttgcaggggaccacgtggggcacgtcggagctgaaagtgctggcaggctcagatgaggactcgatgctgctgcacgggcggtcagagtcagactcctgggccctggccttggccttcaggtgttcctccacgtcacactcgctcgtggactggtaaaagctagtgatggaggagatgggctctatgcttgcggggtcctcttcccactcccaggcatgtagcgacatgctgcagagcgcactgctggccgccggcgctcctgctgacatacctcctctgccaagaagctcactgccttccacagcacatccatcattcttcatcagcagttcctctacccttgagtcttggagacagtgaccttattcccttgtgtcttttcttctccaggctgtagtctggagcctgtggagtagggagatactggcacctccccagtgagatctcaactattatgacctaagctgtagtcacgcggtctcacattgaagcaagaatccccacccgggggttttcacactggttgctgctaagcaacgtgcccattctcggcttgcactgggggaccctgaatgcaggattttatgaatcagagtcatgggctcaaaaaacacgaaattccagggttagccctggctttaggcaaagcctgatccagcagctcaactgatgttactaagggtcctgtttcttttgccgtcatctttgggctctatctgcagcccccaagcatctccggacggccccctcagaggcacaacttcccgcttcgtcggtcatcatgctccgcgccctcaggcagtcagcgaaacgccggaaacgcctgcagacgcctgcagacgctccttgtgtttcattggctacccgtgcagc

SEQ ID NO: 15607 - RNA, 6916 nt, Homo sapiens
  source 1..6916: mol_type = other RNA
gctgggattacaggcatgagccactgtgcccagccctggctgtattcttgaagctgcccggggaaggctcacgaagggaggagcatctggttgtacctgattctggagacagcattttacctgcccctttacccactgtactccatccaaaatgaccctgcagtgccctgcagaggtctcaggccttggcctagagaacagagggctttgctcgtgctccccgctctgtctgcagtgctcttcctcttctatagccactcgaccatatctaggaatgcccagctcagtctacctctgaccctcacagtcctgttgacctgaggttctggatcagtgtccccacaaagcccagtcgtgttgccaagtgatgggtgtaggcgccagcactgtggcacttgctgagagtggcatatgattttttgcaggtcctagccctgggggtagcccagacacccccccagtgctgacaggttatgtgctgtggagggtgctgaaatggtttctcctccagtgggctggaatcacagatgggctgtttacggagcaagtgccggctccaccccatgagatctgggggttagagatgagcaggatgagtcctttgtaactgagaatgaagctgtacccctttctctccctgcagccctgaatcacttgctgggggtctggaggaggggttcacccttagggctgcttcatggtgggtgggctgactttgtggaaaaatgcccccacttcagccatgtttgtcttatcacggtgcagaaagatcacccaccatctctccttttccttcccagatgctccagaaaacctagatgagcagattaagaaagtgtcccagcagatccttgagaagcgagcctatatctgtgcccaccctctggacaggacatgctgaggcaggggacagtgtcccctgctaccgcccgcccctacccatggcccgttgctggatgactgttactcttttttcagaaggtgttgggattatcacaggttaagccttttgttccccgtctgcacctgaagggttgtcgcctggcctgggagagcctcttccaggttttgacctgcaggcagtgctctctaacaggaccatcacagcttctgaactgagccggagagagagaatggaattgctgacccctggaactggcgggtattctggtcattgaggagacaccatagtggaaactggggcttatgctgctgcctccagggtgtgaggtgggtggggacctgtgtcaggtgtggatagccatttctgctcaaccacacattctctaagaaacagcttgaaagctctgtctgggtcattcatttaaactagaagcagaggcacttaaaacatgtaccaggaaccatttaacaaagaatataaaatgtcacaatctgtgtactgttagcctttgctgtacttgtcacactgttccttagaaccagcctttaatgggtgacagcaggaccctgagaaccaccctttggtgatggcctcgggtcccctttgtcctcaccctgcaaggagggcccagaatgctaaggagcagacacacagtgcaggccacaatcccttggggttatgagcccttagtttttatccttctcaggagatgatggggaggctgtctcagctgatgatgttcccacctagggactttagtttctttacaagaactggcttctactcttgaggagaggatgaatggtatctccaggccagcaggcctttgcatttctccagcctcccttctgctggcacttgaaagattacaccaggtcccagcgtgctcactgtggtgaactttaagctttgatgtggtccttgggtggtctggagctctaaaatgcctattgtggacactcccttgagcacagagaaggcagccgactctttttcctccaagtatattcccaatttactgtgatgctggaaataggcaaggaggagactgggaacttggagagctgagctggctgagtggggctggcctgagcattctgccaggggtttggtaactagtttttaaaatggggaaagtttgtaaatattgtgaccgtgtaaataacctctcagtgaaacctgaagttctgttagtgatagcagggcagcattttgcacaaaatgaagcatgcatacctctggacagaaggctgcttagagtttctttgcacaggagaagtttggggaggggctgtcagacccaccccccttctgtgcagccttctggaagggggcttcactctaggctggtggcgtgtaaggcctcagtcttacatgccaatggagaatggcaagttctccattcatccatctgggttgaaaaggcctagcgaccagttcaagcctctccctctcatctgtagttgctaacttttcttaaacatgttgtgggaagaggagaccccagcaagtgtttcttaagtgatttcaccagtgaaacccccaggagacttttgctgggaaggctggcagtggagctcactaggaagccttcttaccaaggaaaagccttgtgttcttaggctagacagctctcctagctggagcctccttgagagccacagcagtaactgtgggcctgggacatgcccacagagagcaggtctcttcaggcaacctgggagatctagggcctactggggagggagggagccaagtctaggcaaatggagaaagtgacatttcagcaaacttgttagcacttccatggagctgtgatcagttgtccttaggagtcgaggaggagaggaagccatcacgttcacctgacctagttttctgggagaagtttctctggcagaccttgtttttagataggctcatgtctctttctccctgaacaaaggttctggctctgttaaccaagtttgggttctatgttaacctccagatgatcctgagatcaattttcataaacagggataaagaggaagaggacttggagggactggtacagcaagacctacgtttcctgtctctgccttaccccaaagaaagaactgtcagtatctttgccgctggaaggtcccagtgaagcccagagcctctgcccccagctcttggctggacacctagagatcagtcatgggtaatagtgttgaagctcaggaagcctttagacctgtcttccaacttccccactttatagccaagaaaccagacccagggcatgaagggatttgcctcaagtcacacaaatgtcacacttggggctagaatcctggtctgagttccagcccagcattcaatctcttttttcagacccattctgcatcttgcttttcttagcatagaaagtttggttgatagtgtaaacaaaatggataccactgaagatgcagagtggcacagagctcctgcctgcccacggcatcaggaggcccagcttggcaaacccttgcctgttacctgttacaggctttggtgcgggcgaagggagcagctcgaggaaaggtggtggtttcttgtacagatcaaagtccacgtggtgcctgtcccagctccacctgtctcgatccaacacaggctccagtacattagcaaacagggagttttccttccactcctcattcagctctttgatgggtggcagcttgagatcctgaaagctgctttcggtgtcgctctgaagacctgtcacttggaatcccctggctgtgagccaggcctggcgggatttcttctgggctttcttctcctcttccttcaagtccaggggctccaccatggctgagaggtaatcctgtgagtacgtgaatctctttcttggctccttggctatctcttgatacagctccttcttggcaagctctgtagaattcatggtctgggtactatagttgtagacggccttgttggcaggggctgaaattttaatcaccttcgccacggacttcggaggcttcttgctgacctggtaggcttctgtgatatttttctggatgaaactgtgctttttgtctttgttcttcataagcatggcactccgccactgcaggtacttctcctggtgggcgtggatctctaaggtgagggtggagttccgactgtggtagtcctcaagattgggggcaggctgaggtggtagggcaaacagtttctcatctgtgagttcttcttgcgaaaggggcatcccaaactcttggctcaagtcttttatcatagcagaggagggcagcaggtccctcaccgtcacgtcccagagggtggtgctgttatagcagatgtcgtggatcctggctagagcctggaagacccgcctccgctcagtgtctcgcaggaagaacaccgcctgctgcagcagcagctccgtgggctggaagaggtgcacgtggtacaggatggcctccaggtccccatagagccggctgcggaacagcagctgtgagttgtacagcaccttgtatttcctgtgttctgacctgggaatccagctttggtggttctcccacagctgcctcaagccttggtcggccaggccttccaggatgaaaaggtgtgtcttcccgtccagcaggtggaagccagtgagcacatccaggtgctgctgctcctggacccgcacacgcaccttgaaggctgacaggatctgctgcagggtcctgacagggtaggagtccaggccgagggccttagcgttgatcatggtgatgtcctgcagcaggctgtggagcagggagaccttcttaaagtcaaagacgaagatgatgcggccaaactgggagcccccaaggtcaggatcagcagctctggccccggccctcagtggcaccgcgatgtccactcgcaacttgagctgggagtcagcctctaggtagttgcccctgggcattgggccgtgctggtggccatctctggggaccccaagccccacaaccttccttctcctgctgtcctggccgcagtgtgtgggctgaacctcacagctgtggatggggacggccagattcaagtacttgtggccaaggaggaggtcagcaaaactgacctgggcgatgccataagggtaccacatcttgttctgggactcaaaggggttgttctctgtctctctgggagagatgagggcctggaagttgaggtatgaatccagagggtcctccccaaacagcacgggcttctgagaacactcctctgacttgcggtcccggtcgtgaacttccaccaccatgggggggccctccaggtattcccttaggtcactggggtgcagtgccccaaggaagatgacgttgatgtcctggaaataaacgtgggttccatggggctcccccttggtcttgtgaactggagtcttatggaactggtacttgcagtacacaggcatgcacagcctctctagttcctgaatgggtacaggctgtgatggaaggcaggaagcacacttgatctttatggtcaggggatttaaatcctgcttttgctcctcggtcatgatcggaacttctgtttttaaagtcaaaaggcaatctaaaatgttggcagacttctcactgccacgactcacgacagtttgccatccggcaaggagcggcatgacggccagctggatggagaaagcgctctgcttcctggggcctgtcagcgtggggtctgcctcttcttctgccaggggcttcttatgtctcctctggattttccttcttccctctgaatctttccctttaatttgagacctttgtctgtctaatatgtttgttaagctgctaagtgattcactctcaattaattccttgatctccatcatgcttgctcctgccaaagaaatggttggtgttcttgaaacactccattgaatcgtggaagaatcgtccattttgagggacttctcatattcctcactgttcttggaagaagtttcgggctctgcttggtgagaaccttgcaaagactttgggtgtttttctgttttttcttgttttcctggcggatgttcctggttcgactcttctctgacaatgttggtattctcaatgccctgttcagataattttctctgatttaaaaccaaatgtctcacttctgacttatgaaaagctcccacgtcgtctgtgaagccggcagtctttaatcggtaatatctgacttttcttgacatcttgtctttagtgttccagagcctcaaggtgattttgtggaaatttattttctttaataattcctttgtcacagtgatattaaaagtctgctcccacgacacccaggctttgtcaccttcgtgccacggcttcacagtctttactcctgactccaggaatactttggccaccattggaaatagcaatatgtcaacttttttaggttcttcatcgtccggcagaaggaaatactcaatgtggtaaaaacgacgcatctttgtaacagaactgtctgttttagggtgtttcttatatttttcaatcaaacttgcatattttcccttctgacccatattcacagggaaggccagtgagatggtgaatttgcaggggaccacgtggggcacgtcggagctgaaagtgctggcaggctcagatgaggactcgatgctgctgcacgggcggtcagagtcagactcctgggccctggccttggccttcaggtgttcctccacgtcacactcgctcgtggactggtaaaagctagtgatggaggagatgggctctatgcttgcggggtcctcttcccactcccaggcatgtagcgacatgctgcagagcgcactgctggccgccggcgctcctgctgacatacctcctctgccaagaagctcactgccttccacagcacatccatcattcttcatcagcagttcctctgagaccacaaacagggcctggcttgtgtcatcttagaaaacagggaagaagccaggcacggtggttcatgcctgtaatcccaacactttgggaggctgagacaggaggatcactt

SEQ ID NO: 15608 - RNA, 7342 nt, Homo sapiens
  source 1..7342: mol_type = other RNA
gctgggattacaggcatgagccactgtgcccagccctggctgtattcttgaagctgcccggggaaggctcacgaagggaggagcatctggttgtacctgattctggagacagcattttacctgcccctttacccactgtactccatccaaaatgaccctgcagtgccctgcagaggtctcaggccttggcctagagaacagagggctttgctcgtgctccccgctctgtctgcagtgctcttcctcttctatagccactcgaccatatctaggaatgcccagctcagtctacctctgaccctcacagtcctgttgacctgaggttctggatcagtgtccccacaaagcccagtcgtgttgccaagtgatgggtgtaggcgccagcactgtggcacttgctgagagtggcatatgattttttgcaggtcctagccctgggggtagcccagacacccccccagtgctgacaggttatgtgctgtggagggtgctgaaatggtttctcctccagtgggctggaatcacagatgggctgtttacggagcaagtgccggctccaccccatgagatctgggggttagagatgagcaggatgagtcctttgtaactgagaatgaagctgtacccctttctctccctgcagccctgaatcacttgctgggggtctggaggaggggttcacccttagggctgcttcatggtgggtgggctgactttgtggaaaaatgcccccacttcagccatgtttgtcttatcacggtgcagaaagatcacccaccatctctccttttccttcccagatgctccagaaaacctagatgagcagattaagaaagtgtcccagcagatccttgagaagcgagcctatatctgtgcccaccctctggacaggacatgctgaggcaggggacagtgtcccctgctaccgcccgcccctacccatggcccgttgctggatgactgttactcttttttcagaaggtgttgggattatcacaggttaagccttttgttccccgtctgcacctgaagggttgtcgcctggcctgggagagcctcttccaggttttgacctgcaggcagtgctctctaacaggaccatcacagcttctgaactgagccggagagagagaatggaattgctgacccctggaactggcgggtattctggtcattgaggagacaccatagtggaaactggggcttatgctgctgcctccagggtgtgaggtgggtggggacctgtgtcaggtgtggatagccatttctgctcaaccacacattctctaagaaacagcttgaaagctctgtctgggtcattcatttaaactagaagcagaggcacttaaaacatgtaccaggaaccatttaacaaagaatataaaatgtcacaatctgtgtactgttagcctttgctgtacttgtcacactgttccttagaaccagcctttaatgggtgacagcaggaccctgagaaccaccctttggtgatggcctcgggtcccctttgtcctcaccctgcaaggagggcccagaatgctaaggagcagacacacagtgcaggccacaatcccttggggttatgagcccttagtttttatccttctcaggagatgatggggaggctgtctcagctgatgatgttcccacctagggactttagtttctttacaagaactggcttctactcttgaggagaggatgaatggtatctccaggccagcaggcctttgcatttctccagcctcccttctgctggcacttgaaagattacaccaggtcccagcgtgctcactgtggtgaactttaagctttgatgtggtccttgggtggtctggagctctaaaatgcctattgtggacactcccttgagcacagagaaggcagccgactctttttcctccaagtatattcccaatttactgtgatgctggaaataggcaaggaggagactgggaacttggagagctgagctggctgagtggggctggcctgagcattctgccaggggtttggtaactagtttttaaaatggggaaagtttgtaaatattgtgaccgtgtaaataacctctcagtgaaacctgaagttctgttagtgatagcagggcagcattttgcacaaaatgaagcatgcatacctctggacagaaggctgcttagagtttctttgcacaggagaagtttggggaggggctgtcagacccaccccccttctgtgcagccttctggaagggggcttcactctaggctggtggcgtgtaaggcctcagtcttacatgccaatggagaatggcaagttctccattcatccatctgggttgaaaaggcctagcgaccagttcaagcctctccctctcatctgtagttgctaacttttcttaaacatgttgtgggaagaggagaccccagcaagtgtttcttaagtgatttcaccagtgaaacccccaggagacttttgctgggaaggctggcagtggagctcactaggaagccttcttaccaaggaaaagccttgtgttcttaggctagacagctctcctagctggagcctccttgagagccacagcagtaactgtgggcctgggacatgcccacagagagcaggtctcttcaggcaacctgggagatctagggcctactggggagggagggagccaagtctaggcaaatggagaaagtgacatttcagcaaacttgttagcacttccatggagctgtgatcagttgtccttaggagtcgaggaggagaggaagccatcacgttcacctgacctagttttctgggagaagtttctctggcagaccttgtttttagataggctcatgtctctttctccctgaacaaaggttctggctctgttaaccaagtttgggttctatgttaacctccagatgatcctgagatcaattttcataaacagggataaagaggaagaggacttggagggactggtacagcaagacctacgtttcctgtctctgccttaccccaaagaaagaactgtcagtatctttgccgctggaaggtcccagtgaagcccagagcctctgcccccagctcttggctggacacctagagatcagtcatgggtaatagtgttgaagctcaggaagcctttagacctgtcttccaacttccccactttatagccaagaaaccagacccagggcatgaagggatttgcctcaagtcacacaaatgtcacacttggggctagaatcctggtctgagttccagcccagcattcaatctcttttttcagacccattctgcatcttgcttttcttagcatagaaagtttggttgatagtgtaaacaaaatggataccactgaagatgcagagtggcacagagctcctgcctgcccacggcatcaggaggcccagcttggcaaacccttgcctgttacctgttacaggctttggtgcgggcgaagggagcagctcgaggaaaggtggtggtttcttgtacagatcaaagtccacgtggtgcctgtcccagctccacctgtctcgatccaacacaggctccagtacattagcaaacagggagttttccttccactcctcattcagctctttgatgggtggcagcttgagatcctgaaagctgctttcggtgtcgctctgaagacctgtcacttggaatcccctggctgtgagccaggcctggcgggatttcttctgggctttcttctcctcttccttcaagtccaggggctccaccatggctgagaggtaatcctgtgagtacgtgaatctctttcttggctccttggctatctcttgatacagctccttcttggcaagctctgtagaattcatggtctgggtactatagttgtagacggccttgttggcaggggctgaaattttaatcaccttcgccacggacttcggaggcttcttgctgacctggtaggcttctgtgatatttttctggatgaaactgtgctttttgtctttgttcttcataagcatggcactccgccactgcaggtacttctcctggtgggcgtggatctctaaggtgagggtggagttccgactgtggtagtcctcaagattgggggcaggctgaggtggtagggcaaacagtttctcatctgtgagttcttcttgcgaaaggggcatcccaaactcttggctcaagtcttttatcatagcagaggagggcagcaggtccctcaccgtcacgtcccagagggtggtgctgttatagcagatgtcgtggatcctggctagagcctggaagacccgcctccgctcagtgtctcgcaggaagaacaccgcctgctgcagcagcagctccgtgggctggaagaggtgcacgtggtacaggatggcctccaggtccccatagagccggctgcggaacagcagctgtgagttgtacagcaccttgtatttcctgtgttctgacctgggaatccagctttggtggttctcccacagctgcctcaagccttggtcggccaggccttccaggatgaaaaggtgtgtcttcccgtccagcaggtggaagccagtgagcacatccaggtgctgctgctcctggacccgcacacgcaccttgaaggctgacaggatctgctgcagggtcctgacagggtaggagtccaggccgagggccttagcgttgatcatggtgatgtcctgcagcaggctgtggagcagggagaccttcttaaagtcaaagacgaagatgatgcggccaaactgggagcccccaaggtcaggatcagcagctctggccccggccctcagtggcaccgcgatgtccactcgcaacttgagctgggagtcagcctctaggtagttgcccctgggcattgggccgtgctggtggccatctctggggaccccaagccccacaaccttccttctcctgctgtcctggccgcagtgtgtgggctgaacctcacagctgtggatggggacggccagattcaagtacttgtggccaaggaggaggtcagcaaaactgacctgggcgatgccataagggtaccacatcttgttctgggactcaaaggggttgttctctgtctctctgggagagatgagggcctggaagttgaggtatgaatccagagggtcctccccaaacagcacgggcttctgagaacactcctctgacttgcggtcccggtcgtgaacttccaccaccatgggggggccctccaggtattcccttaggtcactggggtgcagtgccccaaggaagatgacgttgatgtcctggaaataaacgtgggttccatggggctcccccttggtcttgtgaactggagtcttatggaactggtacttgcagtacacaggcatgcacagcctctctagttcctgaatgggtacaggctgtgatggaaggcaggaagcacacttgatctttatggtcaggggatttaaatcctgcttttgctcctcggtcatgatcggaacttctgtttttaaagtcaaaaggcaatctaaaatgttggcagacttctcactgccacgactcacgacagtttgccatccggcaaggagcggcatgacggccagctggatggagaaagcgctctgcttcctggggcctgtcagcgtggggtctgcctcttcttctgccaggggcttcttatgtctcctctggattttccttcttccctctgaatctttccctttaatttgagacctttgtctgtctaatatgtttgttaagctgctaagtgattcactctcaattaattccttgatctccatcatgcttgctcctgccaaagaaatggttggtgttcttgaaacactccattgaatcgtggaagaatcgtccattttgagggacttctcatattcctcactgttcttggaagaagtttcgggctctgcttggtgagaaccttgcaaagactttgggtgtttttctgttttttcttgttttcctggcggatgttcctggttcgactcttctctgacaatgttggtattctcaatgccctgttcagataattttctctgatttaaaaccaaatgtctcacttctgacttatgaaaagctcccacgtcgtctgtgaagccggcagtctttaatcggtaatatctgacttttcttgacatcttgtctttagtgttccagagcctcaaggtgattttgtggaaatttattttctttaataattcctttgtcacagtgatattaaaagtctgctcccacgacacccaggctttgtcaccttcgtgccacggcttcacagtctttactcctgactccaggaatactttggccaccattggaaatagcaatatgtcaacttttttaggttcttcatcgtccggcagaaggaaatactcaatgtggtaaaaacgacgcatctttgtaacagaactgtctgttttagggtgtttcttatatttttcaatcaaacttgcatattttcccttctgacccatattcacagggaaggccagtgagatggtgaatttgcaggggaccacgtggggcacgtcggagctgaaagtgctggcaggctcagatgaggactcgatgctgctgcacgggcggtcagagtcagactcctgggccctggccttggccttcaggtgttcctccacgtcacactcgctcgtggactggtaaaagctagtgatggaggagatgggctctatgcttgcggggtcctcttcccactcccaggcatgtagcgacatgctgcagagcgcactgctggccgccggcgctcctgctgacatacctcctctgccaagaagctcactgccttccacagcacatccatcattcttcatcagcagttcctgcctctacccttgagtcttggagacagtgaccttattcccttgtgtcttttcttctccaggctgtagtctggagcctgtggagtagggagatactggcacctccccagtgagatctcaactattatgacctaagctgtagtcacgcggtctcacattgaagcaagaatccccacccgggggttttcacactggttgctgctaagcaacgtgcccattctcggcttgcactgggggaccctgaatgcaggattttatgaatcagagtcatgggctcaaaaaacacgaaattccagggttagccctggctttaggcaaagcctgatccagcagctcaactgatgttactaagggtcctgtttcttttgccgtcatctttgggctctatctgcagcccccaagcatctccggacggccccctcagaggcacaacttcccgcttcgtcggtcatcatgctccgcgccctcaggcagtcagcgaaacgccggaaacgcctgcagacgcctgcagacgctccttgtgtttcattggctacccgtgcagc

SEQ ID NO: 15609 - RNA, 7309 nt, Homo sapiens
  source 1..7309: mol_type = other RNA
gctgggattacaggcatgagccactgtgcccagccctggctgtattcttgaagctgcccggggaaggctcacgaagggaggagcatctggttgtacctgattctggagacagcattttacctgcccctttacccactgtactccatccaaaatgaccctgcagtgccctgcagaggtctcaggccttggcctagagaacagagggctttgctcgtgctccccgctctgtctgcagtgctcttcctcttctatagccactcgaccatatctaggaatgcccagctcagtctacctctgaccctcacagtcctgttgacctgaggttctggatcagtgtccccacaaagcccagtcgtgttgccaagtgatgggtgtaggcgccagcactgtggcacttgctgagagtggcatatgattttttgcaggtcctagccctgggggtagcccagacacccccccagtgctgacaggttatgtgctgtggagggtgctgaaatggtttctcctccagtgggctggaatcacagatgggctgtttacggagcaagtgccggctccaccccatgagatctgggggttagagatgagcaggatgagtcctttgtaactgagaatgaagctgtacccctttctctccctgcagccctgaatcacttgctgggggtctggaggaggggttcacccttagggctgcttcatggtgggtgggctgactttgtggaaaaatgcccccacttcagccatgtttgtcttatcacggtgcagaaagatcacccaccatctctccttttccttcccagatgctccagaaaacctagatgagcagattaagaaagtgtcccagcagatccttgagaagcgagcctatatctgtgcccaccctctggacaggacatgctgaggcaggggacagtgtcccctgctaccgcccgcccctacccatggcccgttgctggatgactgttactcttttttcagaaggtgttgggattatcacaggttaagccttttgttccccgtctgcacctgaagggttgtcgcctggcctgggagagcctcttccaggttttgacctgcaggcagtgctctctaacaggaccatcacagcttctgaactgagccggagagagagaatggaattgctgacccctggaactggcgggtattctggtcattgaggagacaccatagtggaaactggggcttatgctgctgcctccagggtgtgaggtgggtggggacctgtgtcaggtgtggatagccatttctgctcaaccacacattctctaagaaacagcttgaaagctctgtctgggtcattcatttaaactagaagcagaggcacttaaaacatgtaccaggaaccatttaacaaagaatataaaatgtcacaatctgtgtactgttagcctttgctgtacttgtcacactgttccttagaaccagcctttaatgggtgacagcaggaccctgagaaccaccctttggtgatggcctcgggtcccctttgtcctcaccctgcaaggagggcccagaatgctaaggagcagacacacagtgcaggccacaatcccttggggttatgagcccttagtttttatccttctcaggagatgatggggaggctgtctcagctgatgatgttcccacctagggactttagtttctttacaagaactggcttctactcttgaggagaggatgaatggtatctccaggccagcaggcctttgcatttctccagcctcccttctgctggcacttgaaagattacaccaggtcccagcgtgctcactgtggtgaactttaagctttgatgtggtccttgggtggtctggagctctaaaatgcctattgtggacactcccttgagcacagagaaggcagccgactctttttcctccaagtatattcccaatttactgtgatgctggaaataggcaaggaggagactgggaacttggagagctgagctggctgagtggggctggcctgagcattctgccaggggtttggtaactagtttttaaaatggggaaagtttgtaaatattgtgaccgtgtaaataacctctcagtgaaacctgaagttctgttagtgatagcagggcagcattttgcacaaaatgaagcatgcatacctctggacagaaggctgcttagagtttctttgcacaggagaagtttggggaggggctgtcagacccaccccccttctgtgcagccttctggaagggggcttcactctaggctggtggcgtgtaaggcctcagtcttacatgccaatggagaatggcaagttctccattcatccatctgggttgaaaaggcctagcgaccagttcaagcctctccctctcatctgtagttgctaacttttcttaaacatgttgtgggaagaggagaccccagcaagtgtttcttaagtgatttcaccagtgaaacccccaggagacttttgctgggaaggctggcagtggagctcactaggaagccttcttaccaaggaaaagccttgtgttcttaggctagacagctctcctagctggagcctccttgagagccacagcagtaactgtgggcctgggacatgcccacagagagcaggtctcttcaggcaacctgggagatctagggcctactggggagggagggagccaagtctaggcaaatggagaaagtgacatttcagcaaacttgttagcacttccatggagctgtgatcagttgtccttaggagtcgaggaggagaggaagccatcacgttcacctgacctagttttctgggagaagtttctctggcagaccttgtttttagataggctcatgtctctttctccctgaacaaaggttctggctctgttaaccaagtttgggttctatgttaacctccagatgatcctgagatcaattttcataaacagggataaagaggaagaggacttggagggactggtacagcaagacctacgtttcctgtctctgccttaccccaaagaaagaactgtcagtatctttgccgctggaaggtcccagtgaagcccagagcctctgcccccagctcttggctggacacctagagatcagtcatgggtaatagtgttgaagctcaggaagcctttagacctgtcttccaacttccccactttatagccaagaaaccagacccagggcatgaagggatttgcctcaagtcacacaaatgtcacacttggggctagaatcctggtctgagttccagcccagcattcaatctcttttttcagacccattctgcatcttgcttttcttagcatagaaagtttggttgatagtgtaaacaaaatggataccactgaagatgcagagtggcacagagctcctgcctgcccacggcatcaggaggcccagcttggcaaacccttgcctgttacctgttacaggctttggtgcgggcgaagggagcagctcgaggaaaggtggtggtttcttgtacagatcaaagtccacgtggtgcctgtcccagctccacctgtctcgatccaacacaggctccagtacattagcaaacagggagttttccttccactcctcattcagctctttgatgggtggcagcttgagatcctgaaagctgctttcggtgtcgctctgaagacctgtcacttggaatcccctggctgtgagccaggcctggcgggatttcttctgggctttcttctcctcttccttcaagtccaggggctccaccatggctgagaggtaatcctgtgagtacgtgaatctctttcttggctccttggctatctcttgatacagctccttcttggcaagctctgtagaattcatggtctgggtactatagttgtagacggccttgttggcaggggctgaaattttaatcaccttcgccacggacttcggaggcttcttgctgacctggtaggcttctgtgatatttttctggatgaaactgtgctttttgtctttgttcttcataagcatggcactccgccactgcaggtacttctcctggtgggcgtggatctctaaggtgagggtggagttccgactgtggtagtcctcaagattgggggcaggctgaggtggtagggcaaacagtttctcatctgtgagttcttcttgcgaaaggggcatcccaaactcttggctcaagtcttttatcatagcagaggagggcagcaggtccctcaccgtcacgtcccagagggtggtgctgttatagcagatgtcgtggatcctggctagagcctggaagacccgcctccgctcagtgtctcgcaggaagaacaccgcctgctgcagcagcagctccgtgggctggaagaggtgcacgtggtacaggatggcctccaggtccccatagagccggctgcggaacagcagctgtgagttgtacagcaccttgtatttcctgtgttctgacctgggaatccagctttggtggttctcccacagctgcctcaagccttggtcggccaggccttccaggatgaaaaggtgtgtcttcccgtccagcaggtggaagccagtgagcacatccaggtgctgctgctcctggacccgcacacgcaccttgaaggctgacaggatctgctgcagggtcctgacagggtaggagtccaggccgagggccttagcgttgatcatggtgatgtcctgcagcaggctgtggagcagggagaccttcttaaagtcaaagacgaagatgatgcggccaaactgggagcccccaaggtcaggatcagcagctctggccccggccctcagtggcaccgcgatgtccactcgcaacttgagctgggagtcagcctctaggtagttgcccctgggcattgggccgtgctggtggccatctctggggaccccaagccccacaaccttccttctcctgctgtcctggccgcagtgtgtgggctgaacctcacagctgtggatggggacggccagattcaagtacttgtggccaaggaggaggtcagcaaaactgacctgggcgatgccataagggtaccacatcttgttctgggactcaaaggggttgttctctgtctctctgggagagatgagggcctggaagttgaggtatgaatccagagggtcctccccaaacagcacgggcttctgagaacactcctctgacttgcggtcccggtcgtgaacttccaccaccatgggggggccctccaggtattcccttaggtcactggggtgcagtgccccaaggaagatgacgttgatgtcctggaaataaacgtgggttccatggggctcccccttggtcttgtgaactggagtcttatggaactggtacttgcagtacacaggcatgcacagcctctctagttcctgaatgggtacaggctgtgatggaaggcaggaagcacacttgatctttatggtcaggggatttaaatcctgcttttgctcctcggtcatgatcggaacttctgtttttaaagtcaaaaggcaatctaaaatgttggcagacttctcactgccacgactcacgacagtttgccatccggcaaggagcggcatgacggccagctggatggagaaagcgctctgcttcctggggcctgtcagcgtggggtctgcctcttcttctgccaggggcttcttatgtctcctctggattttccttcttccctctgaatctttccctttaatttgagacctttgtctgtctaatatgtttgttaagctgctaagtgattcactctcaattaattccttgatctccatcatgcttgctcctgccaaagaaatggttggtgttcttgaaacactccattgaatcgtggaagaatcgtccattttgagggacttctcatattcctcactgttcttggaagaagtttcgggctctgcttggtgagaaccttgcaaagactttgggtgtttttctgttttttcttgttttcctggcggatgttcctggttcgactcttctctgacaatgttggtattctcaatgccctgttcagataattttctctgatttaaaaccaaatgtctcacttctgacttatgaaaagctcccacgtcgtctgtgaagccggcagtctttaatcggtaatatctgacttttcttgacatcttgtctttagtgttccagagcctcaaggtgattttgtggaaatttattttctttaataattcctttgtcacagtgatattaaaagtctgctcccacgacacccaggctttgtcaccttcgtgccacggcttcacagtctttactcctgactccaggaatactttggccaccattggaaatagcaatatgtcaacttttttaggttcttcatcgtccggcagaaggaaatactcaatgtggtaaaaacgacgcatctttgtaacagaactgtctgttttagggtgtttcttatatttttcaatcaaacttgcatattttcccttctgacccatattcacagggaaggccagtgagatggtgaatttgcaggggaccacgtggggcacgtcggagctgaaagtgctggcaggctcagatgaggactcgatgctgctgcacgggcggtcagagtcagactcctgggccctggccttggccttcaggtgttcctccacgtcacactcgctcgtggactggtaaaagctagtgatggaggagatgggctctatgcttgcggggtcctcttcccactcccaggcatgtagcgacatgctgcagagcgcactgctggccgccggcgctcctgctgacatacctcctctgccaagaagctcactgccttccacagcacatccatcattcttcatcagcagttccttattcccttgtgtcttttcttctccaggctgtagtctggagcctgtggagtagggagatactggcacctccccagtgagatctcaactattatgacctaagctgtagtcacgcggtctcacattgaagcaagaatccccacccgggggttttcacactggttgctgctaagcaacgtgcccattctcggcttgcactgggggaccctgaatgcaggattttatgaatcagagtcatgggctcaaaaaacacgaaattccagggttagccctggctttaggcaaagcctgatccagcagctcaactgatgttactaagggtcctgtttcttttgccgtcatctttgggctctatctgcagcccccaagcatctccggacggccccctcagaggcacaacttcccgcttcgtcggtcatcatgctccgcgccctcaggcagtcagcgaaacgccggaaacgcctgcagacgcctgcagacgctccttgtgtttcattggctacccgtgcagc

SEQ ID NO: 15610 - RNA, 11994 nt, Homo sapiens
  source 1..11994: mol_type = other RNA
gctgggattacaggcatgagccactgtgcccagccctggctgtattcttgaagctgcccggggaaggctcacgaagggaggagcatctggttgtacctgattctggagacagcattttacctgcccctttacccactgtactccatccaaaatgaccctgcagtgccctgcagaggtctcaggccttggcctagagaacagagggctttgctcgtgctccccgctctgtctgcagtgctcttcctcttctatagccactcgaccatatctaggaatgcccagctcagtctacctctgaccctcacagtcctgttgacctgaggttctggatcagtgtccccacaaagcccagtcgtgttgccaagtgatgggtgtaggcgccagcactgtggcacttgctgagagtggcatatgattttttgcaggtcctagccctgggggtagcccagacacccccccagtgctgacaggttatgtgctgtggagggtgctgaaatggtttctcctccagtgggctggaatcacagatgggctgtttacggagcaagtgccggctccaccccatgagatctgggggttagagatgagcaggatgagtcctttgtaactgagaatgaagctgtacccctttctctccctgcagccctgaatcacttgctgggggtctggaggaggggttcacccttagggctgcttcatggtgggtgggctgactttgtggaaaaatgcccccacttcagccatgtttgtcttatcacggtgcagaaagatcacccaccatctctccttttccttcccagatgctccagaaaacctagatgagcagattaagaaagtgtcccagcagatccttgagaagcgagcctatatctgtgcccaccctctggacaggacatgctgaggcaggggacagtgtcccctgctaccgcccgcccctacccatggcccgttgctggatgactgttactcttttttcagaaggtgttgggattatcacaggttaagccttttgttccccgtctgcacctgaagggttgtcgcctggcctgggagagcctcttccaggttttgacctgcaggcagtgctctctaacaggaccatcacagcttctgaactgagccggagagagagaatggaattgctgacccctggaactggcgggtattctggtcattgaggagacaccatagtggaaactggggcttatgctgctgcctccagggtgtgaggtgggtggggacctgtgtcaggtgtggatagccatttctgctcaaccacacattctctaagaaacagcttgaaagctctgtctgggtcattcatttaaactagaagcagaggcacttaaaacatgtaccaggaaccatttaacaaagaatataaaatgtcacaatctgtgtactgttagcctttgctgtacttgtcacactgttccttagaaccagcctttaatgggtgacagcaggaccctgagaaccaccctttggtgatggcctcgggtcccctttgtcctcaccctgcaaggagggcccagaatgctaaggagcagacacacagtgcaggccacaatcccttggggttatgagcccttagtttttatccttctcaggagatgatggggaggctgtctcagctgatgatgttcccacctagggactttagtttctttacaagaactggcttctactcttgaggagaggatgaatggtatctccaggccagcaggcctttgcatttctccagcctcccttctgctggcacttgaaagattacaccaggtcccagcgtgctcactgtggtgaactttaagctttgatgtggtccttgggtggtctggagctctaaaatgcctattgtggacactcccttgagcacagagaaggcagccgactctttttcctccaagtatattcccaatttactgtgatgctggaaataggcaaggaggagactgggaacttggagagctgagctggctgagtggggctggcctgagcattctgccaggggtttggtaactagtttttaaaatggggaaagtttgtaaatattgtgaccgtgtaaataacctctcagtgaaacctgaagttctgttagtgatagcagggcagcattttgcacaaaatgaagcatgcatacctctggacagaaggctgcttagagtttctttgcacaggagaagtttggggaggggctgtcagacccaccccccttctgtgcagccttctggaagggggcttcactctaggctggtggcgtgtaaggcctcagtcttacatgccaatggagaatggcaagttctccattcatccatctgggttgaaaaggcctagcgaccagttcaagcctctccctctcatctgtagttgctaacttttcttaaacatgttgtgggaagaggagaccccagcaagtgtttcttaagtgatttcaccagtgaaacccccaggagacttttgctgggaaggctggcagtggagctcactaggaagccttcttaccaaggaaaagccttgtgttcttaggctagacagctctcctagctggagcctccttgagagccacagcagtaactgtgggcctgggacatgcccacagagagcaggtctcttcaggcaacctgggagatctagggcctactggggagggagggagccaagtctaggcaaatggagaaagtgacatttcagcaaacttgttagcacttccatggagctgtgatcagttgtccttaggagtcgaggaggagaggaagccatcacgttcacctgacctagttttctgggagaagtttctctggcagaccttgtttttagataggctcatgtctctttctccctgaacaaaggttctggctctgttaaccaagtttgggttctatgttaacctccagatgatcctgagatcaattttcataaacagggataaagaggaagaggacttggagggactggtacagcaagacctacgtttcctgtctctgccttaccccaaagaaagaactgtcagtatctttgccgctggaaggtcccagtgaagcccagagcctctgcccccagctcttggctggacacctagagatcagtcatgggtaatagtgttgaagctcaggaagcctttagacctgtcttccaacttccccactttatagccaagaaaccagacccagggcatgaagggatttgcctcaagtcacacaaatgtcacacttggggctagaatcctggtctgagttccagcccagcattcaatctcttttttcagacccattctgcatcttgcttttcttagcatagaaagtttggttgatagtgtaaacaaaatggataccactgaagatgcagagtggcacagagctcctgcctgcccacggcatcaggaggcccagcttggcaaacccttgcctgttacctgttacaggctttggtgcgggcgaagggagcagctcgaggaaaggtggtggtttcttgtacagatcaaagtccacgtggtgcctgtcccagctccacctgtctcgatccaacacaggctccagtacattagcaaacagggagttttccttccactcctcattcagctctttgatgggtggcagcttgagatcctgaaagctgctttcggtgtcgctctgaagacctgtcacttggaatcccctggctgtgagccaggcctggcgggatttcttctgggctttcttctcctcttccttcaagtccaggggctccaccatggctgagaggtaatcctgtgagtacgtgaatctctttcttggctccttggctatctcttgatacagctccttcttggcaagctctgtagaattcatggtctgggtactatagttgtagacggccttgttggcaggggctgaaattttaatcaccttcgccacggacttcggaggcttcttgctgacctggtaggcttctgtgatatttttctggatgaaactgtgctttttgtctttgttcttcataagcatggcactccgccactgcaggtacttctcctggtgggcgtggatctctaaggtgagggtggagttccgactgtggtagtcctcaagattgggggcaggctgaggtggtagggcaaacagtttctcatctgtgagttcttcttgcgaaaggggcatcccaaactcttggctcaagtcttttatcatagcagaggagggcagcaggtccctcaccgtcacgtcccagagggtggtgctgttatagcagatgtcgtggatcctggctagagcctggaagacccgcctccgctcagtgtctcgcaggaagaacaccgcctgctgcagcagcagctccgtgggctggaagaggtgcacgtggtacaggatggcctccaggtccccatagagccggctgcggaacagcagctgtgagttgtacagcaccttgtatttcctgtgttctgacctgggaatccagctttggtggttctcccacagctgcctcaagccttggtcggccaggccttccaggatgaaaaggtgtgtcttcccgtccagcaggtggaagccagtgagcacatccaggtgctgctgctcctggacccgcacacgcaccttgaaggctgacaggatctgctgcagggtcctgacagggtaggagtccaggccgagggccttagcgttgatcatggtgatgtcctgcagcaggctgtggagcagggagaccttcttaaagtcaaagacgaagatgatgcggccaaactgggagcccccaaggtcaggatcagcagctctggccccggccctcagtggcaccgcgatgtccactcgcaacttgagctgggagtcagcctctaggtagttgcccctgggcattgggccgtgctggtggccatctctggggaccccaagccccacaaccttccttctcctgctgtcctggccgcagtgtgtgggctgaacctcacagctgtggatggggacggccagattcaagtacttgtggccaaggaggaggtcagcaaaactgacctgggcgatgccataagggtaccacatcttgttctgggactcaaaggggttgttctctgtctctctgggagagatgagggcctggaagttgaggtatgaatccagagggtcctccccaaacagcacgggcttctgagaacactcctctgacttgcggtcccggtcgtgaacttccaccaccatgggggggccctccaggtattcccttaggtcactggggtgcagtgccccaaggaagatgacgttgatgtcctggaaataaacgtgggttccatggggctcccccttggtcttgtgaactggagtcttatggaactggtacttgcagtacacaggcatgcacagcctctctagttcctgaatgggtacaggctgtgatggaaggcaggaagcacacttgatctttatggtcaggggatttaaatcctgcttttgctcctcggtcatgatcggaacttctgtttttaaagtcaaaaggcaatctaaaatgttggcagacttctcactgccacgactcacgacagtttgccatccggcaaggagcggcatgacggccagctggatggagaaagcgctctgcttcctggggcctgtcagcgtggggtctgcctcttcttctgccaggggcttcttatgtctcctctggattttccttcttccctctgaatctttccctttaatttgagacctttgtctgtctaatatgtttgttaagctgctaagtgattcactctcaattaattccttgatctccatcatgcttgctcctgccaaagaaatggttggtgttcttgaaacactccattgaatcgtggaagaatcgtccattttgagggacttctcatattcctcactgttcttggaagaagtttcgggctctgcttggtgagaaccttgcaaagactttgggtgtttttctgttttttcttgttttcctggcggatgttcctggttcgactcttctctgacaatgttggtattctcaatgccctgttcagataattttctctgatttaaaaccaaatgtctcacttctgacttatgaaaagctcccacgtcgtctgtgaagccggcagtctttaatcggtaatatctgacttttcttgacatcttgtctttagtgttccagagcctcaaggtgattttgtggaaatttattttctttaataattcctttgtcacagtgatattaaaagtctgctcccacgacacccaggctttgtcaccttcgtgccacggcttcacagtctttactcctgactccaggaatactttggccaccattggaaatagcaatatgtcaacttttttaggttcttcatcgtccggcagaaggaaatactcaatgtggtaaaaacgacgcatctttgtaacagaactgtctgttttagggtgtttcttatatttttcaatcaaacttgcatattttcccttctgacctgcgagcggatgcgctgggcggcagcggggagttggaccgcggcggcaactcccgtaccggatccacagccacctgggcgaagagactccaagactgagaggagcgtccgccggtgcagggagggccgcaggcccagccactcagctacgtttggcggttgctaggagacgcgagggcgtgcggcctgggggcggggctccgcggggcggggctttccccctcagccactgcgcgcagtttgtcaaatggctacatccaggttcagaaaccagctgccttcattccttcactcatgcattcactcattaaggagtttctactcggaacgtcagcacctactataagcctggtccttgcccgtacgatgggaggtaggggttgatggctccttcctccccctccatcagctcccacctcccattctttaataaaagcaaaggaagctgtgggctctgcaaactccagacctccccacgatccctctcattagattctctgcttctgtcgccgatgtccttaaaaaccagacctccccacgatccctctcattagattctctgcttctgtcgctgatgtccttaaaatagcatgagaattcttgttagtgatcatgagcgccaactcagagatcagaaaacaaagcttagagaggtgaagcgattcgcccgaggtcacacagcaagtagggcgcagcactgtgttgaaatccggactgcctgactccaaagcctccgctcgtctgctaaaccacccaagctgagagccctggctgcggctcctaatgtagaggacctcagcacagcaagcggctgggacagagggctggggtaggcctcatggaggaagtgagcaacgccaaatctggggggtgactaggcagaggcggtgaaagcaagagaaagcatcccaggtagaggaacagcatatgcaaaggcccatagaggtgaaagggcatggcaagtttcaggaatgggtggcgaggctgtagcagtgtgcagggcccatggtacatagccccacagggcaggttagggcacaggactatgggcaatggggagccaaggcaggtcttctgttgagggagggcaccctgctccggcagtcagtttgttcaagagaatgggagctgaggctacacacaagcttggctattaagaaaactttagctgagttgagctatgacctactttgtgtcaaagagcaaaactgtggcgcagctggggctgagacccaagtcctgagcctcccagtgcatgcctccccagaccgctctcagggcatgggacagcccctttaatactgggtgctccaatactcctcgggttcagtctgaaaaacagcctcaagtacagctgttagggaagacaccaaatggcagtgggccctgtgaggagtgggttcaaactcttagcacgagaacggcaaccaccttgcccacaccccacctgcagcagcctggagactgctgtctgtatgccaggaagtgctcaggagacacatgaagggctggaagaatacaaagctactcagatacaccagcccccaaaagggccctttaacaagggcagttcaacactaccaccactcttggacagacatcaggcctcctgctccccaggtcctacccactggcctgaggctggtttccctccaaaggttcctagatcacatcaccacctaggacagaagccaatctcttcccaagctcaatagtgagaggccagaggtcttggaccaagggccaatgtgccatcctggatgtgcactggaaacacctacatgtcaaaaatacaattctgaggcttcattaaagacctgtggaagtgactctccaggggtggagcttagaaaccagtggcagattgtattttccaaagacagccacctcaaaagatcccctcccacataatcttccggcaggcattgtgaggttcacattcctcccacccagttggggggtctagtctccttctctggaaactgggcagacctctgtgactggctcagtcaaaagagtgcagaggaaatgacactatgtgatttctgaggccaggtcatataaattccatctacctctgccctgttcttttgaggtatagtattcatgctaggaatccagctagcatgttgtgaggaagcccaagcagccatgtgaaatggccacatgaaactgttgtgactgacggttcccagccaattgcagcctcaacccccagacatatgagagtgcaagacttcaaatgatcccagccctcagtctttgagccaccctggctgacattgaggaacagaaacaagctgtctccatcatgagaaattgtagatttataagcaaattgttgctctcttaaaccactaagttttggggtgatttgttgtgcaataaataataggaacgggagccatatttttaaattaccaccaagattgtattgcacaaccagaatatggaaccactgccctgagagagatggtgtctgggtcaagacctagggcatcacaggatgaagtgagggcaaaggtgtgctacccactactcaggtatgagacagtggtgggtctacaaccctacctcagtgaagatggcttcagggctggcagatcagaagcaaaggaaggggggcttctgtttcagttatctgttactgagtaaaaaccatccccaaacttaatggtgtcaaacaaacacttgttatttctcaccactccatgcatcagctgagtagttctctgctggcctcgcctgggctcactccctatgctgtgctcagctggaggaccaacatggctggaagctgccagaagtcctcacttgcatgtctggcagttgctgctggctcttcgtgggcccgctggttcccctccatgggttcccccgcccccagtggtacaccagcttccttctatgtggtgcctcatctcctcatagcccggcctggcttcctcagatggcattctcagagcagggatcccagagggcaaagaagaagttgcaaggcctcttgggacctaggcgtggaaccagcaccatgtcactctgctacatgccattaaccaaagcaagtcatgaggctggccccacttcaaggggatgaagacatggactgtacatctggtaagcagagggacaagcatccaggggcaggaggtgttcaaggtcactgaacaatccatcccttcatccttactctgccgggtggagggttcccaagctcccacaggctatgtagaggccttcctgaagctatcccaagactctggcagctggaagcatattgggaatcagctacatacaccttcttcttgccccttccccatttttaacagctttattgaagtattttttatttaataaaatccatccatttcaagcgtagaattcaatgattttcagtaactttacctagtgctgtaatcatcatcataaattcattttagaacattttcatccccctaataagacttcatgcacatttataattaatctctgttccaactcccagtcctaggcaaccatatctactttgtttctaaaaattggccttttctagacatttcctataaattgagtcagacactgtgttctggctttgtgactggtttctttcacctaccgttatgtttccaaggtttatttatgttgaggcatgtgtcagtatttcattccttttcatgactgaataatattctattgtatggacagaccacagtttgcctatccattcatcagttaatgggcatttggcttgggcatttagacatttatgaacaacgttgctatgaacattcccacacaagtctttgtgtggatgtgttttcatctctcttgggtcgatatctaggagtggaagagttgggtcgtatggtcattttgtgattaacttcttgagaaactgccaaactatcttccacaggggctgcatcattttgtgttcccatcaacaacatgaagtttcctgtttctccaaattcttgacaagatttattgcctgttttattcactacagctattctcatgagtataatatagtatttcatcatagttttcatgtgcatttccctaacaagaatactgagattgttttatgcacatgttggctatttatacaacttctttggtgaaatgtctgtttgtatcttcacccactttttgattggattgtttgtcttcttgttactgagttgttaagagttcattgtaaattcggaatataagtcctttactgggcatatgttttacaaatattttctcctagtctcttgttcgtcatattttcttaatagtgtcttttgaagtgcaaatgttttgaactttgatgaaggtccgattcatcatttttttcttttttggatcatgcatttggtgtcgtatctaagaaatctttgactaacaacaggcctatttttaatagaagtaaagcttggtgtctgaacactaagcaaatctactaaccaagacccctaaaaacccaaaagctttatgacactgaaaataatggcccaaggacattcccagacagttctgggctctggatagaacaacacaagtttccaaaaaacaggctgataataccacaagcttataaaatatgtatactccttggcccagtaataaatcactcaagatatggcacaaactgttcacagtatggtttttgcggagaaaagctgaaaaccacctcagtgggcatctgtgggggatgacaaagcaccttatagttcatccccagggagcacagagcagcctctggagcagtgtctgcaaagaaaccacagccaagctgtttacaaagctcagttcctgtgcaaagaaagatcccaatggcgccctttccactgtgcttttcatgtcaagttgaatgagctacgatttgcacactgtaaaattcagatgtacacagtcatgcaaccactacaccatgaagatagagtatttcaatcactccaaaaagttctttcatgcccaaatacatagaaaagtctggaaataaatacatcagaaatacacagtgatcctctcttggtggcagaatggtggatgatttttgctttttagcattttcccggacctttaaaagacactttaaacaatatactatttgaaatggctcaaacaatactgaactgacttcagaaaatcatttctttgccacagccctgactctctcccacacagacacacgcccatccccccagctcatacaaaagaacgcaaggagacctctgagtttgctcactttgaaccttaaacaaaaaccttgtggatgcaaccagaattatttcagaggtgcctggtaacaccgcagggcagacagacaggcctgacagcaaaccattatcaacccttacttccctgagctgtaggggagtggaggccggcaacggctcccagcaagacatttaaaagctttcttttcaatattgactggcccaggaaagctactgttcaaaggattccttcaccagctgcagggatggggggtggggagggtgttgcactcttgcctgggctaccagctcttagggctgacatgaaataaaatcaggttctttttttttttt

SEQ ID NO: 15611 - RNA, 6499 nt, Homo sapiens
  source 1..6499: mol_type = other RNA
gctgggattacaggcatgagccactgtgcccagccctggctgtattcttgaagctgcccggggaaggctcacgaagggaggagcatctggttgtacctgattctggagacagcattttacctgcccctttacccactgtactccatccaaaatgaccctgcagtgccctgcagaggtctcaggccttggcctagagaacagagggctttgctcgtgctccccgctctgtctgcagtgctcttcctcttctatagccactcgaccatatctaggaatgcccagctcagtctacctctgaccctcacagtcctgttgacctgaggttctggatcagtgtccccacaaagcccagtcgtgttgccaagtgatgggtgtaggcgccagcactgtggcacttgctgagagtggcatatgattttttgcaggtcctagccctgggggtagcccagacacccccccagtgctgacaggttatgtgctgtggagggtgctgaaatggtttctcctccagtgggctggaatcacagatgggctgtttacggagcaagtgccggctccaccccatgagatctgggggttagagatgagcaggatgagtcctttgtaactgagaatgaagctgtacccctttctctccctgcagccctgaatcacttgctgggggtctggaggaggggttcacccttagggctgcttcatggtgggtgggctgactttgtggaaaaatgcccccacttcagccatgtttgtcttatcacggtgcagaaagatcacccaccatctctccttttccttcccagatgctccagaaaacctagatgagcagattaagaaagtgtcccagcagatccttgagaagcgagcctatatctgtgcccaccctctggacaggacatgctgaggcaggggacagtgtcccctgctaccgcccgcccctacccatggcccgttgctggatgactgttactcttttttcagaaggtgttgggattatcacaggttaagccttttgttccccgtctgcacctgaagggttgtcgcctggcctgggagagcctcttccaggttttgacctgcaggcagtgctctctaacaggaccatcacagcttctgaactgagccggagagagagaatggaattgctgacccctggaactggcgggtattctggtcattgaggagacaccatagtggaaactggggcttatgctgctgcctccagggtgtgaggtgggtggggacctgtgtcaggtgtggatagccatttctgctcaaccacacattctctaagaaacagcttgaaagctctgtctgggtcattcatttaaactagaagcagaggcacttaaaacatgtaccaggaaccatttaacaaagaatataaaatgtcacaatctgtgtactgttagcctttgctgtacttgtcacactgttccttagaaccagcctttaatgggtgacagcaggaccctgagaaccaccctttggtgatggcctcgggtcccctttgtcctcaccctgcaaggagggcccagaatgctaaggagcagacacacagtgcaggccacaatcccttggggttatgagcccttagtttttatccttctcaggagatgatggggaggctgtctcagctgatgatgttcccacctagggactttagtttctttacaagaactggcttctactcttgaggagaggatgaatggtatctccaggccagcaggcctttgcatttctccagcctcccttctgctggcacttgaaagattacaccaggtcccagcgtgctcactgtggtgaactttaagctttgatgtggtccttgggtggtctggagctctaaaatgcctattgtggacactcccttgagcacagagaaggcagccgactctttttcctccaagtatattcccaatttactgtgatgctggaaataggcaaggaggagactgggaacttggagagctgagctggctgagtggggctggcctgagcattctgccaggggtttggtaactagtttttaaaatggggaaagtttgtaaatattgtgaccgtgtaaataacctctcagtgaaacctgaagttctgttagtgatagcagggcagcattttgcacaaaatgaagcatgcatacctctggacagaaggctgcttagagtttctttgcacaggagaagtttggggaggggctgtcagacccaccccccttctgtgcagccttctggaagggggcttcactctaggctggtggcgtgtaaggcctcagtcttacatgccaatggagaatggcaagttctccattcatccatctgggttgaaaaggcctagcgaccagttcaagcctctccctctcatctgtagttgctaacttttcttaaacatgttgtgggaagaggagaccccagcaagtgtttcttaagtgatttcaccagtgaaacccccaggagacttttgctgggaaggctggcagtggagctcactaggaagccttcttaccaaggaaaagccttgtgttcttaggctagacagctctcctagctggagcctccttgagagccacagcagtaactgtgggcctgggacatgcccacagagagcaggtctcttcaggcaacctgggagatctagggcctactggggagggagggagccaagtctaggcaaatggagaaagtgacatttcagcaaacttgttagcacttccatggagctgtgatcagttgtccttaggagtcgaggaggagaggaagccatcacgttcacctgacctagttttctgggagaagtttctctggcagaccttgtttttagataggctcatgtctctttctccctgaacaaaggttctggctctgttaaccaagtttgggttctatgttaacctccagatgatcctgagatcaattttcataaacagggataaagaggaagaggacttggagggactggtacagcaagacctacgtttcctgtctctgccttaccccaaagaaagaactgtcagtatctttgccgctggaaggtcccagtgaagcccagagcctctgcccccagctcttggctggacacctagagatcagtcatgggtaatagtgttgaagctcaggaagcctttagacctgtcttccaacttccccactttatagccaagaaaccagacccagggcatgaagggatttgcctcaagtcacacaaatgtcacacttggggctagaatcctggtctgagttccagcccagcattcaatctcttttttcagacccattctgcatcttgcttttcttagcatagaaagtttggttgatagtgtaaacaaaatggataccactgaagatgcagagtggcacagagctcctgcctgcccacggcatcaggaggcccagcttggcaaacccttgcctgttacctgttacaggctttggtgcgggcgaagggagcagctcgaggaaaggtggtggtttcttgtacagatcaaagtccacgtggtgcctgtcccagctccacctgtctcgatccaacacaggctccagtacattagcaaacagggagttttccttccactcctcattcagctctttgatgggtggcagcttgagatcctgaaagctgctttcggtgtcgctctgaagacctgtcacttggaatcccctggctgtgagccaggcctggcgggatttcttctgggctttcttctcctcttccttcaagtccaggggctccaccatggctgagaggtaatcctgtgagtacgtgaatctctttcttggctccttggctatctcttgatacagctccttcttggcaagctctgtagaattcatggtctgggtactatagttgtagacggccttgttggcaggggctgaaattttaatcaccttcgccacggacttcggaggcttcttgctgacctggtaggcttctgtgatatttttctggatgaaactgtgctttttgtctttgttcttcataagcatggcactccgccactgcaggtacttctcctggtgggcgtggatctctaaggtgagggtggagttccgactgtggtagtcctcaagattgggggcaggctgaggtggtagggcaaacagtttctcatctgtgagttcttcttgcgaaaggggcatcccaaactcttggctcaagtcttttatcatagcagaggagggcagcaggtccctcaccgtcacgtcccagagggtggtgctgttatagcagatgtcgtggatcctggctagagcctggaagacccgcctccgctcagtgtctcgcaggaagaacaccgcctgctgcagcagcagctccgtgggctggaagaggtgcacgtggtacaggatggcctccaggtccccatagagccggctgcggaacagcagctgtgagttgtacagcaccttgtatttcctgtgttctgacctgggaatccagctttggtggttctcccacagctgcctcaagccttggtcggccaggccttccaggatgaaaaggtgtgtcttcccgtccagcaggtggaagccagtgagcacatccaggtgctgctgctcctggacccgcacacgcaccttgaaggctgacaggatctgctgcagggtcctgacagggtaggagtccaggccgagggccttagcgttgatcatggtgatgtcctgcagcaggctgtggagcagggagaccttcttaaagtcaaagacgaagatgatgcggccaaactgggagcccccaaggtcaggatcagcagctctggccccggccctcagtggcaccgcgatgtccactcgcaacttgagctgggagtcagcctctaggtagttgcccctgggcattgggccgtgctggtggccatctctggggaccccaagccccacaaccttccttctcctgctgtcctggccgcagtgtgtgggctgaacctcacagctgtggatggggacggccagattcaagtacttgtggccaaggaggaggtcagcaaaactgacctgggcgatgccataagggtaccacatcttgttctgggactcaaaggggttgttctctgtctctctgggagagatgagggcctggaagttgaggtatgaatccagagggtcctccccaaacagcacgggcttctgagaacactcctctgacttgcggtcccggtcgtgaacttccaccaccatgggggggccctccaggtattcccttaggtcactggggtgcagtgccccaaggaagatgacgttgatgtcctggaaataaacgtgggttccatggggctcccccttggtcttgtgaactggagtcttatggaactggtacttgcagtacacaggcatgcacagcctctctagttcctgaatgggtacaggctgtgatggaaggcaggaagcacacttgatctttatggtcaggggatttaaatcctgcttttgctcctcggtcatgatcggaacttctgtttttaaagtcaaaaggcaatctaaaatgttggcagacttctcactgccacgactcacgacagtttgccatccggcaaggagcggcatgacggccagctggatggagaaagcgctctgcttcctggggcctgtcagcgtggggtctgcctcttcttctgccaggggcttcttatgtctcctctggattttccttcttccctctgaatctttccctttaatttgagacctttgtctgtctaatatgtttgttaagctgctaagtgattcactctcaattaattccttgatctccatcatgcttgctcctgccaaagaaatggttggtgttcttgaaacactccattgaatcgtggaagaatcgtccattttgagggacttctcatattcctcactgttcttggaagaagtttcgggctctgcttggtgagaaccttgcaaagactttgggtgtttttctgttttttcttgttttcctggcggatgttcctggttcgactcttctctgacaatgttggtattctcaatgccctgttcagataattttctctgatttaaaaccaaatgtctcacttctgacttatgaaaagctcccacgtcgtctgtgaagccggcagtctttaatcggtaatatctgacttttcttgacatcttgtctttagtgttccagagcctcaaggtgattttgtggaaatttattttctttaataattcctttgtcacagtgatattaaaagtctgctcccacgacacccaggctttgtcaccttcgtgccacggcttcacagtctttactcctgactccaggaatactttggccaccattggaaatagcaatatgtcaacttttttaggttcttcatcgtccggcagaaggaaatactcaatgtggtaaaaacgacgcatctttgtaacagaactgtctgttttagggtgtttcttatatttttcaatcaaacttgcatattttcccttctgacctgctgacatacctcctctgccaagaagctcactgccttccacagcacatccatcattcttcatcagca

SEQ ID NO: 15612 - RNA, 6560 nt, Homo sapiens
  source 1..6560: mol_type = other RNA
gctgggattacaggcatgagccactgtgcccagccctggctgtattcttgaagctgcccggggaaggctcacgaagggaggagcatctggttgtacctgattctggagacagcattttacctgcccctttacccactgtactccatccaaaatgaccctgcagtgccctgcagaggtctcaggccttggcctagagaacagagggctttgctcgtgctccccgctctgtctgcagtgctcttcctcttctatagccactcgaccatatctaggaatgcccagctcagtctacctctgaccctcacagtcctgttgacctgaggttctggatcagtgtccccacaaagcccagtcgtgttgccaagtgatgggtgtaggcgccagcactgtggcacttgctgagagtggcatatgattttttgcaggtcctagccctgggggtagcccagacacccccccagtgctgacaggttatgtgctgtggagggtgctgaaatggtttctcctccagtgggctggaatcacagatgggctgtttacggagcaagtgccggctccaccccatgagatctgggggttagagatgagcaggatgagtcctttgtaactgagaatgaagctgtacccctttctctccctgcagccctgaatcacttgctgggggtctggaggaggggttcacccttagggctgcttcatggtgggtgggctgactttgtggaaaaatgcccccacttcagccatgtttgtcttatcacggtgcagaaagatcacccaccatctctccttttccttcccagatgctccagaaaacctagatgagcagattaagaaagtgtcccagcagatccttgagaagcgagcctatatctgtgcccaccctctggacaggacatgctgaggcaggggacagtgtcccctgctaccgcccgcccctacccatggcccgttgctggatgactgttactcttttttcagaaggtgttgggattatcacaggttaagccttttgttccccgtctgcacctgaagggttgtcgcctggcctgggagagcctcttccaggttttgacctgcaggcagtgctctctaacaggaccatcacagcttctgaactgagccggagagagagaatggaattgctgacccctggaactggcgggtattctggtcattgaggagacaccatagtggaaactggggcttatgctgctgcctccagggtgtgaggtgggtggggacctgtgtcaggtgtggatagccatttctgctcaaccacacattctctaagaaacagcttgaaagctctgtctgggtcattcatttaaactagaagcagaggcacttaaaacatgtaccaggaaccatttaacaaagaatataaaatgtcacaatctgtgtactgttagcctttgctgtacttgtcacactgttccttagaaccagcctttaatgggtgacagcaggaccctgagaaccaccctttggtgatggcctcgggtcccctttgtcctcaccctgcaaggagggcccagaatgctaaggagcagacacacagtgcaggccacaatcccttggggttatgagcccttagtttttatccttctcaggagatgatggggaggctgtctcagctgatgatgttcccacctagggactttagtttctttacaagaactggcttctactcttgaggagaggatgaatggtatctccaggccagcaggcctttgcatttctccagcctcccttctgctggcacttgaaagattacaccaggtcccagcgtgctcactgtggtgaactttaagctttgatgtggtccttgggtggtctggagctctaaaatgcctattgtggacactcccttgagcacagagaaggcagccgactctttttcctccaagtatattcccaatttactgtgatgctggaaataggcaaggaggagactgggaacttggagagctgagctggctgagtggggctggcctgagcattctgccaggggtttggtaactagtttttaaaatggggaaagtttgtaaatattgtgaccgtgtaaataacctctcagtgaaacctgaagttctgttagtgatagcagggcagcattttgcacaaaatgaagcatgcatacctctggacagaaggctgcttagagtttctttgcacaggagaagtttggggaggggctgtcagacccaccccccttctgtgcagccttctggaagggggcttcactctaggctggtggcgtgtaaggcctcagtcttacatgccaatggagaatggcaagttctccattcatccatctgggttgaaaaggcctagcgaccagttcaagcctctccctctcatctgtagttgctaacttttcttaaacatgttgtgggaagaggagaccccagcaagtgtttcttaagtgatttcaccagtgaaacccccaggagacttttgctgggaaggctggcagtggagctcactaggaagccttcttaccaaggaaaagccttgtgttcttaggctagacagctctcctagctggagcctccttgagagccacagcagtaactgtgggcctgggacatgcccacagagagcaggtctcttcaggcaacctgggagatctagggcctactggggagggagggagccaagtctaggcaaatggagaaagtgacatttcagcaaacttgttagcacttccatggagctgtgatcagttgtccttaggagtcgaggaggagaggaagccatcacgttcacctgacctagttttctgggagaagtttctctggcagaccttgtttttagataggctcatgtctctttctccctgaacaaaggttctggctctgttaaccaagtttgggttctatgttaacctccagatgatcctgagatcaattttcataaacagggataaagaggaagaggacttggagggactggtacagcaagacctacgtttcctgtctctgccttaccccaaagaaagaactgtcagtatctttgccgctggaaggtcccagtgaagcccagagcctctgcccccagctcttggctggacacctagagatcagtcatgggtaatagtgttgaagctcaggaagcctttagacctgtcttccaacttccccactttatagccaagaaaccagacccagggcatgaagggatttgcctcaagtcacacaaatgtcacacttggggctagaatcctggtctgagttccagcccagcattcaatctcttttttcagacccattctgcatcttgcttttcttagcatagaaagtttggttgatagtgtaaacaaaatggataccactgaagatgcagagtggcacagagctcctgcctgcccacggcatcaggaggcccagcttggcaaacccttgcctgttacctgttacaggctttggtgcgggcgaagggagcagctcgaggaaaggtggtggtttcttgtacagatcaaagtccacgtggtgcctgtcccagctccacctgtctcgatccaacacaggctccagtacattagcaaacagggagttttccttccactcctcattcagctctttgatgggtggcagcttgagatcctgaaagctgctttcggtgtcgctctgaagacctgtcacttggaatcccctggctgtgagccaggcctggcgggatttcttctgggctttcttctcctcttccttcaagtccaggggctccaccatggctgagaggtaatcctgtgagtacgtgaatctctttcttggctccttggctatctcttgatacagctccttcttggcaagctctgtagaattcatggtctgggtactatagttgtagacggccttgttggcaggggctgaaattttaatcaccttcgccacggacttcggaggcttcttgctgacctggtaggcttctgtgatatttttctggatgaaactgtgctttttgtctttgttcttcataagcatggcactccgccactgcaggtacttctcctggtgggcgtggatctctaaggtgagggtggagttccgactgtggtagtcctcaagattgggggcaggctgaggtggtagggcaaacagtttctcatctgtgagttcttcttgcgaaaggggcatcccaaactcttggctcaagtcttttatcatagcagaggagggcagcaggtccctcaccgtcacgtcccagagggtggtgctgttatagcagatgtcgtggatcctggctagagcctggaagacccgcctccgctcagtgtctcgcaggaagaacaccgcctgctgcagcagcagctccgtgggctggaagaggtgcacgtggtacaggatggcctccaggtccccatagagccggctgcggaacagcagctgtgagttgtacagcaccttgtatttcctgtgttctgacctgggaatccagctttggtggttctcccacagctgcctcaagccttggtcggccaggccttccaggatgaaaaggtgtgtcttcccgtccagcaggtggaagccagtgagcacatccaggtgctgctgctcctggacccgcacacgcaccttgaaggctgacaggatctgctgcagggtcctgacagggtaggagtccaggccgagggccttagcgttgatcatggtgatgtcctgcagcaggctgtggagcagggagaccttcttaaagtcaaagacgaagatgatgcggccaaactgggagcccccaaggtcaggatcagcagctctggccccggccctcagtggcaccgcgatgtccactcgcaacttgagctgggagtcagcctctaggtagttgcccctgggcattgggccgtgctggtggccatctctggggaccccaagccccacaaccttccttctcctgctgtcctggccgcagtgtgtgggctgaacctcacagctgtggatggggacggccagattcaagtacttgtggccaaggaggaggtcagcaaaactgacctgggcgatgccataagggtaccacatcttgttctgggactcaaaggggttgttctctgtctctctgggagagatgagggcctggaagttgaggtatgaatccagagggtcctccccaaacagcacgggcttctgagaacactcctctgacttgcggtcccggtcgtgaacttccaccaccatgggggggccctccaggtattcccttaggtcactggggtgcagtgccccaaggaagatgacgttgatgtcctggaaataaacgtgggttccatggggctcccccttggtcttgtgaactggagtcttatggaactggtacttgcagtacacaggcatgcacagcctctctagttcctgaatgggtacaggctgtgatggaaggcaggaagcacacttgatctttatggtcaggggatttaaatcctgcttttgctcctcggtcatgatcggaacttctgtttttaaagtcaaaaggcaatctaaaatgttggcagacttctcactgccacgactcacgacagtttgccatccggcaaggagcggcatgacggccagctggatggagaaagcgctctgcttcctggggcctgtcagcgtggggtctgcctcttcttctgccaggggcttcttatgtctcctctggattttccttcttccctctgaatctttccctttaatttgagacctttgtctgtctaatatgtttgttaagctgctaagtgattcactctcaattaattccttgatctccatcatgcttgctcctgccaaagaaatggttggtgttcttgaaacactccattgaatcgtggaagaatcgtccattttgagggacttctcatattcctcactgttcttggaagaagtttcgggctctgcttggtgagaaccttgcaaagactttgggtgtttttctgttttttcttgttttcctggcggatgttcctggttcgactcttctctgacaatgttggtattctcaatgccctgttcagataattttctctgatttaaaaccaaatgtctcacttctgacttatgaaaagctcccacgtcgtctgtgaagccggcagtctttaatcggtaatatctgacttttcttgacatcttgtctttagtgttccagagcctcaaggtgattttgtggaaatttattttctttaataattcctttgtcacagtgatattaaaagtctgctcccacgacacccaggctttgtcaccttcgtgccacggcttcacagtctttactcctgactccaggaatactttggccaccattggaaatagcaatatgtcaacttttttaggttcttcatcgtccggcagaaggaaatactcaatgtggtaaaaacgacgcatctttgtaacagaactgtctgttttagggtgtttcttatatttttcaatcaaacttgcatattttcccttctgacgtcagcagcgtgcaccagcaaaatagcagaagcaggaggagagccggctggaatacacctaccccatattcacagggaaggccagtgagatggtgaatttgcaggggaccacgtggggcacgtcggagct

SEQ ID NO: 15613 - RNA, 3097 nt, Homo sapiens
  source 1..3097: mol_type = other RNA
gctgggattacaggcatgagccactgtgcccagccgaggtcagcttttatagctgcaaaaatttagtggcaaccataatgggaatagtcattttaaagtcattaaatatgtcatgaaaataataaaaatctatatttactgaaatggcactcatgaaatctttggcatgataaaagcagttaagggtacagcatgcatatcataattacactttcttaaaaaagcaaagtatagcacgattttctctaccaaattgagagcagccatctataagtatgattacaattaattttggctttttagtttgtaattttttgctttgtgattttggcttaacaattaaaaatgtacatttgtaaaataaaaagaccggccgcagtggctcacgcctgtaatcccagcactttcggaggccgaggcgggtggatcacctgaagtcgggagattgagaccatcctggctaacatggtgaaaccccgtctctactaaaaatacaaaaaattagccgggtgttgtggcacatgcctgtaatcccaactactcaaaaggctgaggcagaagaaccacttgaacctgggaggcgaaggttgtgacgagccgagattgcaccattgcactccagcctaggcaacaagagcgaaactccgtctcaacaaaaaataaagccaggtgcaatcgctcatgcctgtaatcccagcactttgggaggctgaggcaggtggatcacctgaggtcaggagttcaagactatcctgaccaacatggagaaaccctgtctctactaaaaatagaaaattagcagggtgtggtggcacacgcctgtgatcccagctactcaggagtctgaggcaggagaattgcttgaagccgggaggtggaggttgcagcgagccgagattgcgccactgcactccagcctgggcaacagagtgaaactccgtctcaaaaaacatataataataataataaaataaaacaaaaagactaacactaacttcaaaaacaaagttaaacctccacaaggaatttaaaaatattaaaggtcacacaattcaaacagtgtgatactggtgcaaacacaaatacacagatcagaaaagatagctctaaaaacacaagcaaatataaacatgagtataatgtgtcaccaagaaagtagaacaaaacaatgaatgaaagaattatagaacagctggcatcggtatatgactgggggagagagggaatgtcactttagactccgaatttataacctggaatgaaatacatttggatacaaaatttaaatacaaagttttaaaaaaaactacggaagagggtaactattagacatgatttttggtttaaaatatgaggaaggtgacaggggctttaatttttattatttattagtatgaattccctgatgacgaatgagatccgagccactactaaaagccttcccacattccttacagttatagggcttttcaccagtgtgaattctcagatgtcgagtaaggtttgagcatttattaaaggcctttccacattcattacattcatatggtttttcatctgtatgaattctctgatgctggaaaagttgtgagttctgagtaaaggccttcccacattcaagacattcaaagggtttctcaccagcgtgaattctctgatgttgacgaagctgtgagctctgagtaaaagcctttccacattccttacaatcatagggtttctcaccagtgtgaattctctgatgattagtaagtgctgagccactactaaaggctttgccacattccttgcactcatagggtttctcaccagtatgaattctctgatgttgaacaagctttgagctctgggtaaaggctttgccacattccttacattcatagggtttctcacctgtatgaattcgtgcatgctgaaaaagttgtgagctcttagtaaaggctttcccacatactttacattcataaggtttttcaccagtgtgaattcgctgatggtcaataagatttgagcaataactaaaggccttcccacattccttacattcatagggtttcttaccggtatggattctctgatgttgagaaaggtatgagctacaactgaaggcctttccacattccttacattcaaagggtttttcgccagtatgaattttcagatgccgagtaacatgtgaaccacaactaaagaatttcccacactctttacattcataagatttttcaccaatatgaattctctgatgttgaataaattgtgagttctgactaaaggcctttccacatttcttacattcatagggtctgtcttcattattaattatttgatggagagtaaggaatgtctgttgaataaatgtgggcatgtattcaggagtgaatatttcttgactaaaatgcccatttggatatcccagttgttttgcaaggtggcttctatattccaaaacatctccaaaactggagtactcaaggccatgctttgtaagtcccattatctccctctggcataattctatttcataaacttccttctttagagataataacttggtttcacacatcgattccagatctgaacacaggcctcttgtaagctctctgccaaccatccagggctctttcccttgttccaataaggagatcacttgaggcttaggagtgtaaagtcccattgaaaccagattgccgtagttctccaacatcacatctctgtataagtccctctgaacagggtccaggcagtcccactcctcctgagagaagtctatggacacatcactgaacatcactgatccctcagccatggcttctagtattgcagatggttagtcttccttgaggccgttctcagaggtatctaaggtagtcaaactcatagaaacagaaagtagaacagtggctgccaggggctgtaatcccagctactcaggaggctgaggcaagagaatcgcttgaacccggaaagcagaggctgcagtgagctgagatcatgccactgcactccagcttgggcaacagagtgagactccgtctgcgggccccagccgagcctgcaagacccaggccgctcaccgcgcacttcccctaccctt

SEQ ID NO: 15614 - RNA, 3067 nt, Homo sapiens
  source 1..3067: mol_type = other RNA
gctgggattacaggcatgagccactgtgcccagccgaggtcagcttttatagctgcaaaaatttagtggcaaccataatgggaatagtcattttaaagtcattaaatatgtcatgaaaataataaaaatctatatttactgaaatggcactcatgaaatctttggcatgataaaagcagttaagggtacagcatgcatatcataattacactttcttaaaaaagcaaagtatagcacgattttctctaccaaattgagagcagccatctataagtatgattacaattaattttggctttttagtttgtaattttttgctttgtgattttggcttaacaattaaaaatgtacatttgtaaaataaaaagaccggccgcagtggctcacgcctgtaatcccagcactttcggaggccgaggcgggtggatcacctgaagtcgggagattgagaccatcctggctaacatggtgaaaccccgtctctactaaaaatacaaaaaattagccgggtgttgtggcacatgcctgtaatcccaactactcaaaaggctgaggcagaagaaccacttgaacctgggaggcgaaggttgtgacgagccgagattgcaccattgcactccagcctaggcaacaagagcgaaactccgtctcaacaaaaaataaagccaggtgcaatcgctcatgcctgtaatcccagcactttgggaggctgaggcaggtggatcacctgaggtcaggagttcaagactatcctgaccaacatggagaaaccctgtctctactaaaaatagaaaattagcagggtgtggtggcacacgcctgtgatcccagctactcaggagtctgaggcaggagaattgcttgaagccgggaggtggaggttgcagcgagccgagattgcgccactgcactccagcctgggcaacagagtgaaactccgtctcaaaaaacatataataataataataaaataaaacaaaaagactaacactaacttcaaaaacaaagttaaacctccacaaggaatttaaaaatattaaaggtcacacaattcaaacagtgtgatactggtgcaaacacaaatacacagatcagaaaagatagctctaaaaacacaagcaaatataaacatgagtataatgtgtcaccaagaaagtagaacaaaacaatgaatgaaagaattatagaacagctggcatcggtatatgactgggggagagagggaatgtcactttagactccgaatttataacctggaatgaaatacatttggatacaaaatttaaatacaaagttttaaaaaaaactacggaagagggtaactattagacatgatttttggtttaaaatatgaggaaggtgacaggggctttaatttttattatttattagtatgaattccctgatgacgaatgagatccgagccactactaaaagccttcccacattccttacagttatagggcttttcaccagtgtgaattctcagatgtcgagtaaggtttgagcatttattaaaggcctttccacattcattacattcatatggtttttcatctgtatgaattctctgatgctggaaaagttgtgagttctgagtaaaggccttcccacattcaagacattcaaagggtttctcaccagcgtgaattctctgatgttgacgaagctgtgagctctgagtaaaagcctttccacattccttacaatcatagggtttctcaccagtgtgaattctctgatgattagtaagtgctgagccactactaaaggctttgccacattccttgcactcatagggtttctcaccagtatgaattctctgatgttgaacaagctttgagctctgggtaaaggctttgccacattccttacattcatagggtttctcacctgtatgaattcgtgcatgctgaaaaagttgtgagctcttagtaaaggctttcccacatactttacattcataaggtttttcaccagtgtgaattcgctgatggtcaataagatttgagcaataactaaaggccttcccacattccttacattcatagggtttcttaccggtatggattctctgatgttgagaaaggtatgagctacaactgaaggcctttccacattccttacattcaaagggtttttcgccagtatgaattttcagatgccgagtaacatgtgaaccacaactaaagaatttcccacactctttacattcataagatttttcaccaatatgaattctctgatgttgaataaattgtgagttctgactaaaggcctttccacatttcttacattcatagggtctgtcttcattattaattatttgatggagagtaaggaatgtctgttgaataaatgtgggcatgtattcaggagtgaatatttcttgactaaaatgcccatttggatatcccagttgttttgcaaggtggcttctatattccaaaacatctccaaaactggagtactcaaggccatgctttgtaagtcccattatctccctctggcataattctatttcataaacttccttctttagagataataacttggtttcacacatcgattccagatctgaacacaggcctcttgtaagctctctgccaaccatccagggctctttcccttgttccaataaggagatcacttgaggcttaggagtgtaaagtcccattgaaaccagattgccgtagttctccaacatcacatctctgtataagtccctctgaacagggtccaggcagtcccactcctcctgagagaagtctatggacacatcactgaacatcactgatccctcagccatggcttctagtattgcagatggttagtcttccttgaggccgttctcatgtctgttgaagtataaaaagggactcagtctcatgatcaacagcttaggaaacttaaatgcacattgctaagtgaaagaagccaattcaaaaagactacatactgtatgattacaacattctggaaaaggcaaaactatggagacaataaaaagattaggagttgacagggagggaggatcagtcagggcacagaggccttttagagcaat

SEQ ID NO: 15615 - RNA, 3267 nt, Homo sapiens
  source 1..3267: mol_type = other RNA
gctgggattacaggcatgagccactgtgcccagccgaggtcagcttttatagctgcaaaaatttagtggcaaccataatgggaatagtcattttaaagtcattaaatatgtcatgaaaataataaaaatctatatttactgaaatggcactcatgaaatctttggcatgataaaagcagttaagggtacagcatgcatatcataattacactttcttaaaaaagcaaagtatagcacgattttctctaccaaattgagagcagccatctataagtatgattacaattaattttggctttttagtttgtaattttttgctttgtgattttggcttaacaattaaaaatgtacatttgtaaaataaaaagaccggccgcagtggctcacgcctgtaatcccagcactttcggaggccgaggcgggtggatcacctgaagtcgggagattgagaccatcctggctaacatggtgaaaccccgtctctactaaaaatacaaaaaattagccgggtgttgtggcacatgcctgtaatcccaactactcaaaaggctgaggcagaagaaccacttgaacctgggaggcgaaggttgtgacgagccgagattgcaccattgcactccagcctaggcaacaagagcgaaactccgtctcaacaaaaaataaagccaggtgcaatcgctcatgcctgtaatcccagcactttgggaggctgaggcaggtggatcacctgaggtcaggagttcaagactatcctgaccaacatggagaaaccctgtctctactaaaaatagaaaattagcagggtgtggtggcacacgcctgtgatcccagctactcaggagtctgaggcaggagaattgcttgaagccgggaggtggaggttgcagcgagccgagattgcgccactgcactccagcctgggcaacagagtgaaactccgtctcaaaaaacatataataataataataaaataaaacaaaaagactaacactaacttcaaaaacaaagttaaacctccacaaggaatttaaaaatattaaaggtcacacaattcaaacagtgtgatactggtgcaaacacaaatacacagatcagaaaagatagctctaaaaacacaagcaaatataaacatgagtataatgtgtcaccaagaaagtagaacaaaacaatgaatgaaagaattatagaacagctggcatcggtatatgactgggggagagagggaatgtcactttagactccgaatttataacctggaatgaaatacatttggatacaaaatttaaatacaaagttttaaaaaaaactacggaagagggtaactattagacatgatttttggtttaaaatatgaggaaggtgacaggggctttaatttttattatttattagtatgaattccctgatgacgaatgagatccgagccactactaaaagccttcccacattccttacagttatagggcttttcaccagtgtgaattctcagatgtcgagtaaggtttgagcatttattaaaggcctttccacattcattacattcatatggtttttcatctgtatgaattctctgatgctggaaaagttgtgagttctgagtaaaggccttcccacattcaagacattcaaagggtttctcaccagcgtgaattctctgatgttgacgaagctgtgagctctgagtaaaagcctttccacattccttacaatcatagggtttctcaccagtgtgaattctctgatgattagtaagtgctgagccactactaaaggctttgccacattccttgcactcatagggtttctcaccagtatgaattctctgatgttgaacaagctttgagctctgggtaaaggctttgccacattccttacattcatagggtttctcacctgtatgaattcgtgcatgctgaaaaagttgtgagctcttagtaaaggctttcccacatactttacattcataaggtttttcaccagtgtgaattcgctgatggtcaataagatttgagcaataactaaaggccttcccacattccttacattcatagggtttcttaccggtatggattctctgatgttgagaaaggtatgagctacaactgaaggcctttccacattccttacattcaaagggtttttcgccagtatgaattttcagatgccgagtaacatgtgaaccacaactaaagaatttcccacactctttacattcataagatttttcaccaatatgaattctctgatgttgaataaattgtgagttctgactaaaggcctttccacatttcttacattcatagggtctgtcttcattattaattatttgatggagagtaaggaatgtctgttgaataaatgtgggcatgtattcaggagtgaatatttcttgactaaaatgcccatttggatatcccagttgttttgcaaggtggcttctatattccaaaacatctccaaaactggagtactcaaggccatgctttgtaagtcccattatctccctctggcataattctatttcataaacttccttctttagagataataacttggtttcacacatcgattccagatctgaacacaggcctcttgtaagctctctgccaaccatccagggctctttcccttgttccaataaggagatcacttgaggcttaggagtgtaaagtcccattgaaaccagattgccgtagttctccaacatcacatctctgtataagtccctctgaacagggtccaggcagtcccactcctcctgagagaagtctatggacacatcactgaacatcactgatccctcagccatggcttctagtattgcagatggttagtcttccttgaggccgttctccgatcactggagatgactctcactccataccctgcccctttgccttatacacaataaataacagcgcgaccaggcattcggggccaataccggtctctgtgtcttggtgatagtggtccctcaggcccagctgtcttttcttctatctctgtcttgggtctttatttctacaatctctcgtctccacacacaaagagaaaatcccacaggccctgcagggctggtatcgcctgtaatcccagctactcaggaggctgaggcaagagaatcgcttgaacccggaaagcagaggctgcagtgagctgagatcatgccactgcactccagcttgggcaacagagtgagactccgtctgcgggccccagccgagcctgcaagacccaggccgctcaccgcgcacttcccctaccctt

SEQ ID NO: 15616 - RNA, 3055 nt, Homo sapiens
  source 1..3055: mol_type = other RNA
gctgggattacaggcatgagccactgtgcccagccgaggtcagcttttatagctgcaaaaatttagtggcaaccataatgggaatagtcattttaaagtcattaaatatgtcatgaaaataataaaaatctatatttactgaaatggcactcatgaaatctttggcatgataaaagcagttaagggtacagcatgcatatcataattacactttcttaaaaaagcaaagtatagcacgattttctctaccaaattgagagcagccatctataagtatgattacaattaattttggctttttagtttgtaattttttgctttgtgattttggcttaacaattaaaaatgtacatttgtaaaataaaaagaccggccgcagtggctcacgcctgtaatcccagcactttcggaggccgaggcgggtggatcacctgaagtcgggagattgagaccatcctggctaacatggtgaaaccccgtctctactaaaaatacaaaaaattagccgggtgttgtggcacatgcctgtaatcccaactactcaaaaggctgaggcagaagaaccacttgaacctgggaggcgaaggttgtgacgagccgagattgcaccattgcactccagcctaggcaacaagagcgaaactccgtctcaacaaaaaataaagccaggtgcaatcgctcatgcctgtaatcccagcactttgggaggctgaggcaggtggatcacctgaggtcaggagttcaagactatcctgaccaacatggagaaaccctgtctctactaaaaatagaaaattagcagggtgtggtggcacacgcctgtgatcccagctactcaggagtctgaggcaggagaattgcttgaagccgggaggtggaggttgcagcgagccgagattgcgccactgcactccagcctgggcaacagagtgaaactccgtctcaaaaaacatataataataataataaaataaaacaaaaagactaacactaacttcaaaaacaaagttaaacctccacaaggaatttaaaaatattaaaggtcacacaattcaaacagtgtgatactggtgcaaacacaaatacacagatcagaaaagatagctctaaaaacacaagcaaatataaacatgagtataatgtgtcaccaagaaagtagaacaaaacaatgaatgaaagaattatagaacagctggcatcggtatatgactgggggagagagggaatgtcactttagactccgaatttataacctggaatgaaatacatttggatacaaaatttaaatacaaagttttaaaaaaaactacggaagagggtaactattagacatgatttttggtttaaaatatgaggaaggtgacaggggctttaatttttattatttattagtatgaattccctgatgacgaatgagatccgagccactactaaaagccttcccacattccttacagttatagggcttttcaccagtgtgaattctcagatgtcgagtaaggtttgagcatttattaaaggcctttccacattcattacattcatatggtttttcatctgtatgaattctctgatgctggaaaagttgtgagttctgagtaaaggccttcccacattcaagacattcaaagggtttctcaccagcgtgaattctctgatgttgacgaagctgtgagctctgagtaaaagcctttccacattccttacaatcatagggtttctcaccagtgtgaattctctgatgattagtaagtgctgagccactactaaaggctttgccacattccttgcactcatagggtttctcaccagtatgaattctctgatgttgaacaagctttgagctctgggtaaaggctttgccacattccttacattcatagggtttctcacctgtatgaattcgtgcatgctgaaaaagttgtgagctcttagtaaaggctttcccacatactttacattcataaggtttttcaccagtgtgaattcgctgatggtcaataagatttgagcaataactaaaggccttcccacattccttacattcatagggtttcttaccggtatggattctctgatgttgagaaaggtatgagctacaactgaaggcctttccacattccttacattcaaagggtttttcgccagtatgaattttcagatgccgagtaacatgtgaaccacaactaaagaatttcccacactctttacattcataagatttttcaccaatatgaattctctgatgttgaataaattgtgagttctgactaaaggcctttccacatttcttacattcatagggtctgtcttcattattaattatttgatggagagtaaggaatgtctgttgaataaatgtgggcatgtattcaggagtgaatatttcttgactaaaatgcccatttggatatcccagttgttttgcaaggtggcttctatattccaaaacatctccaaaactggagtactcaaggccatgctttgtaagtcccattatctccctctggcataattctatttcataaacttccttctttagagataataacttggtttcacacatcgattccagatctgaacacaggcctcttgtaagctctctgccaaccatccagggctctttcccttgttccaataaggagatcacttgaggcttaggagtgtaaagtcccattgaaaccagattgccgtagttctccaacatcacatctctgtataagtccctctgaacagggtccaggcagtcccactcctcctgagagaagtctatggacacatcactgaacatcactgatccctcagccatggcttctagtattgcagatggttagtcttccttgaggccgttctcctgaaaaaggacagtgttctgtaatcccagctactcaggaggctgaggcaagagaatcgcttgaacccggaaagcagaggctgcagtgagctgagatcatgccactgcactccagcttgggcaacagagtgagactccgtctgcgggccccagccgagcctgcaagacccaggccgctcaccgcgcacttcccctaccctt

SEQ ID NO: 15617 - RNA, 2915 nt, Homo sapiens
  source 1..2915: mol_type = other RNA
gctgggattacaggcatgagccactgtgcccagccgaggtcagcttttatagctgcaaaaatttagtggcaaccataatgggaatagtcattttaaagtcattaaatatgtcatgaaaataataaaaatctatatttactgaaatggcactcatgaaatctttggcatgataaaagcagttaagggtacagcatgcatatcataattacactttcttaaaaaagcaaagtatagcacgattttctctaccaaattgagagcagccatctataagtatgattacaattaattttggctttttagtttgtaattttttgctttgtgattttggcttaacaattaaaaatgtacatttgtaaaataaaaagaccggccgcagtggctcacgcctgtaatcccagcactttcggaggccgaggcgggtggatcacctgaagtcgggagattgagaccatcctggctaacatggtgaaaccccgtctctactaaaaatacaaaaaattagccgggtgttgtggcacatgcctgtaatcccaactactcaaaaggctgaggcagaagaaccacttgaacctgggaggcgaaggttgtgacgagccgagattgcaccattgcactccagcctaggcaacaagagcgaaactccgtctcaacaaaaaataaagccaggtgcaatcgctcatgcctgtaatcccagcactttgggaggctgaggcaggtggatcacctgaggtcaggagttcaagactatcctgaccaacatggagaaaccctgtctctactaaaaatagaaaattagcagggtgtggtggcacacgcctgtgatcccagctactcaggagtctgaggcaggagaattgcttgaagccgggaggtggaggttgcagcgagccgagattgcgccactgcactccagcctgggcaacagagtgaaactccgtctcaaaaaacatataataataataataaaataaaacaaaaagactaacactaacttcaaaaacaaagttaaacctccacaaggaatttaaaaatattaaaggtcacacaattcaaacagtgtgatactggtgcaaacacaaatacacagatcagaaaagatagctctaaaaacacaagcaaatataaacatgagtataatgtgtcaccaagaaagtagaacaaaacaatgaatgaaagaattatagaacagctggcatcggtatatgactgggggagagagggaatgtcactttagactccgaatttataacctggaatgaaatacatttggatacaaaatttaaatacaaagttttaaaaaaaactacggaagagggtaactattagacatgatttttggtttaaaatatgaggaaggtgacaggggctttaatttttattatttattagtatgaattccctgatgacgaatgagatccgagccactactaaaagccttcccacattccttacagttatagggcttttcaccagtgtgaattctcagatgtcgagtaaggtttgagcatttattaaaggcctttccacattcattacattcatatggtttttcatctgtatgaattctctgatgctggaaaagttgtgagttctgagtaaaggccttcccacattcaagacattcaaagggtttctcaccagcgtgaattctctgatgttgacgaagctgtgagctctgagtaaaagcctttccacattccttacaatcatagggtttctcaccagtgtgaattctctgatgattagtaagtgctgagccactactaaaggctttgccacattccttgcactcatagggtttctcaccagtatgaattctctgatgttgaacaagctttgagctctgggtaaaggctttgccacattccttacattcatagggtttctcacctgtatgaattcgtgcatgctgaaaaagttgtgagctcttagtaaaggctttcccacatactttacattcataaggtttttcaccagtgtgaattcgctgatggtcaataagatttgagcaataactaaaggccttcccacattccttacattcatagggtttcttaccggtatggattctctgatgttgagaaaggtatgagctacaactgaaggcctttccacattccttacattcaaagggtttttcgccagtatgaattttcagatgccgagtaacatgtgaaccacaactaaagaatttcccacactctttacattcataagatttttcaccaatatgaattctctgatgttgaataaattgtgagttctgactaaaggcctttccacatttcttacattcatagggtctgtcttcattattaattatttgatggagagtaaggaatgtctgttgaataaatgtgggcatgtattcaggagtgaatatttcttgactaaaatgcccatttggatatcccagttgttttgcaaggtggcttctatattccaaaacatctccaaaactggagtactcaaggccatgctttgtaagtcccattatctccctctggcataattctatttcataaacttccttctttagagataataacttggtttcacacatcgattccagatctgaacacaggcctcttgtaagctctctgccaaccatccagggctctttcccttgttccaataaggagatcacttgaggcttaggagtgtaaagtcccattgaaaccagattgccgtagttctccaacatcacatctctgtataagtccctctgaacagggtccaggcagtcccactcctcctgagagaagtctatggacacatcactgaacatcactgatccctcagccatggcttctagtattgcagatggttagtcttccttgaggccgttctcctgcgggccccagccgagcctgcaagacccaggccgctcaccgcgcacttcccctaccctt

SEQ ID NO: 15618 - RNA, 3037 nt, Homo sapiens
  source 1..3037: mol_type = other RNA
gctgggattacaggcatgagccactgtgcccagccgaggtcagcttttatagctgcaaaaatttagtggcaaccataatgggaatagtcattttaaagtcattaaatatgtcatgaaaataataaaaatctatatttactgaaatggcactcatgaaatctttggcatgataaaagcagttaagggtacagcatgcatatcataattacactttcttaaaaaagcaaagtatagcacgattttctctaccaaattgagagcagccatctataagtatgattacaattaattttggctttttagtttgtaattttttgctttgtgattttggcttaacaattaaaaatgtacatttgtaaaataaaaagaccggccgcagtggctcacgcctgtaatcccagcactttcggaggccgaggcgggtggatcacctgaagtcgggagattgagaccatcctggctaacatggtgaaaccccgtctctactaaaaatacaaaaaattagccgggtgttgtggcacatgcctgtaatcccaactactcaaaaggctgaggcagaagaaccacttgaacctgggaggcgaaggttgtgacgagccgagattgcaccattgcactccagcctaggcaacaagagcgaaactccgtctcaacaaaaaataaagccaggtgcaatcgctcatgcctgtaatcccagcactttgggaggctgaggcaggtggatcacctgaggtcaggagttcaagactatcctgaccaacatggagaaaccctgtctctactaaaaatagaaaattagcagggtgtggtggcacacgcctgtgatcccagctactcaggagtctgaggcaggagaattgcttgaagccgggaggtggaggttgcagcgagccgagattgcgccactgcactccagcctgggcaacagagtgaaactccgtctcaaaaaacatataataataataataaaataaaacaaaaagactaacactaacttcaaaaacaaagttaaacctccacaaggaatttaaaaatattaaaggtcacacaattcaaacagtgtgatactggtgcaaacacaaatacacagatcagaaaagatagctctaaaaacacaagcaaatataaacatgagtataatgtgtcaccaagaaagtagaacaaaacaatgaatgaaagaattatagaacagctggcatcggtatatgactgggggagagagggaatgtcactttagactccgaatttataacctggaatgaaatacatttggatacaaaatttaaatacaaagttttaaaaaaaactacggaagagggtaactattagacatgatttttggtttaaaatatgaggaaggtgacaggggctttaatttttattatttattagtatgaattccctgatgacgaatgagatccgagccactactaaaagccttcccacattccttacagttatagggcttttcaccagtgtgaattctcagatgtcgagtaaggtttgagcatttattaaaggcctttccacattcattacattcatatggtttttcatctgtatgaattctctgatgctggaaaagttgtgagttctgagtaaaggccttcccacattcaagacattcaaagggtttctcaccagcgtgaattctctgatgttgacgaagctgtgagctctgagtaaaagcctttccacattccttacaatcatagggtttctcaccagtgtgaattctctgatgattagtaagtgctgagccactactaaaggctttgccacattccttgcactcatagggtttctcaccagtatgaattctctgatgttgaacaagctttgagctctgggtaaaggctttgccacattccttacattcatagggtttctcacctgtatgaattcgtgcatgctgaaaaagttgtgagctcttagtaaaggctttcccacatactttacattcataaggtttttcaccagtgtgaattcgctgatggtcaataagatttgagcaataactaaaggccttcccacattccttacattcatagggtttcttaccggtatggattctctgatgttgagaaaggtatgagctacaactgaaggcctttccacattccttacattcaaagggtttttcgccagtatgaattttcagatgccgagtaacatgtgaaccacaactaaagaatttcccacactctttacattcataagatttttcaccaatatgaattctctgatgttgaataaattgtgagttctgactaaaggcctttccacatttcttacattcatagggtctgtcttcattattaattatttgatggagagtaaggaatgtctgttgaataaatgtgggcatgtattcaggagtgaatatttcttgactaaaatgcccatttggatatcccagttgttttgcaaggtggcttctatattccaaaacatctccaaaactggagtactcaaggccatgctttgtaagtcccattatctccctctggcataattctatttcataaacttccttctttagagataataacttggtttcacacatcgattccagatctgaacacaggcctcttgtaagctctctgccaaccatccagggctctttcccttgttccaataaggagatcacttgaggcttaggagtgtaaagtcccattgaaaccagattgccgtagttctccaacatcacatctctgtataagtccctctgaacagggtccaggcagtcccactcctcctgagagaagtctatggacacatcactgaacatcactgatccctcagccatggcttctagtattgcagatggttagtcttccttgaggccgttctcctgtaatcccagctactcaggaggctgaggcaagagaatcgcttgaacccggaaagcagaggctgcagtgagctgagatcatgccactgcactccagcttgggcaacagagtgagactccgtctgcgggccccagccgagcctgcaagacccaggccgctcaccgcgcacttcccctaccctt

SEQ ID NO: 15619 - RNA, 3262 nt, Homo sapiens
  source 1..3262: mol_type = other RNA
gctgggattacaggcatgagccactgtgcccagccgaggtcagcttttatagctgcaaaaatttagtggcaaccataatgggaatagtcattttaaagtcattaaatatgtcatgaaaataataaaaatctatatttactgaaatggcactcatgaaatctttggcatgataaaagcagttaagggtacagcatgcatatcataattacactttcttaaaaaagcaaagtatagcacgattttctctaccaaattgagagcagccatctataagtatgattacaattaattttggctttttagtttgtaattttttgctttgtgattttggcttaacaattaaaaatgtacatttgtaaaataaaaagaccggccgcagtggctcacgcctgtaatcccagcactttcggaggccgaggcgggtggatcacctgaagtcgggagattgagaccatcctggctaacatggtgaaaccccgtctctactaaaaatacaaaaaattagccgggtgttgtggcacatgcctgtaatcccaactactcaaaaggctgaggcagaagaaccacttgaacctgggaggcgaaggttgtgacgagccgagattgcaccattgcactccagcctaggcaacaagagcgaaactccgtctcaacaaaaaataaagccaggtgcaatcgctcatgcctgtaatcccagcactttgggaggctgaggcaggtggatcacctgaggtcaggagttcaagactatcctgaccaacatggagaaaccctgtctctactaaaaatagaaaattagcagggtgtggtggcacacgcctgtgatcccagctactcaggagtctgaggcaggagaattgcttgaagccgggaggtggaggttgcagcgagccgagattgcgccactgcactccagcctgggcaacagagtgaaactccgtctcaaaaaacatataataataataataaaataaaacaaaaagactaacactaacttcaaaaacaaagttaaacctccacaaggaatttaaaaatattaaaggtcacacaattcaaacagtgtgatactggtgcaaacacaaatacacagatcagaaaagatagctctaaaaacacaagcaaatataaacatgagtataatgtgtcaccaagaaagtagaacaaaacaatgaatgaaagaattatagaacagctggcatcggtatatgactgggggagagagggaatgtcactttagactccgaatttataacctggaatgaaatacatttggatacaaaatttaaatacaaagttttaaaaaaaactacggaagagggtaactattagacatgatttttggtttaaaatatgaggaaggtgacaggggctttaatttttattatttattagtatgaattccctgatgacgaatgagatccgagccactactaaaagccttcccacattccttacagttatagggcttttcaccagtgtgaattctcagatgtcgagtaaggtttgagcatttattaaaggcctttccacattcattacattcatatggtttttcatctgtatgaattctctgatgctggaaaagttgtgagttctgagtaaaggccttcccacattcaagacattcaaagggtttctcaccagcgtgaattctctgatgttgacgaagctgtgagctctgagtaaaagcctttccacattccttacaatcatagggtttctcaccagtgtgaattctctgatgattagtaagtgctgagccactactaaaggctttgccacattccttgcactcatagggtttctcaccagtatgaattctctgatgttgaacaagctttgagctctgggtaaaggctttgccacattccttacattcatagggtttctcacctgtatgaattcgtgcatgctgaaaaagttgtgagctcttagtaaaggctttcccacatactttacattcataaggtttttcaccagtgtgaattcgctgatggtcaataagatttgagcaataactaaaggccttcccacattccttacattcatagggtttcttaccggtatggattctctgatgttgagaaaggtatgagctacaactgaaggcctttccacattccttacattcaaagggtttttcgccagtatgaattttcagatgccgagtaacatgtgaaccacaactaaagaatttcccacactctttacattcataagatttttcaccaatatgaattctctgatgttgaataaattgtgagttctgactaaaggcctttccacatttcttacattcatagggtctgtcttcattattaattatttgatggagagtaaggaatgtctgttgaataaatgtgggcatgtattcaggagtgaatatttcttgactaaaatgcccatttggatatcccagttgttttgcaaggtggcttctatattccaaaacatctccaaaactggagtactcaaggccatgctttgtaagtcccattatctccctctggcataattctatttcataaacttccttctttagagataataacttggtttcacacatcgattccagatctgaacacaggcctcttgtaagctctctgccaaccatccagggctctttcccttgttccaataaggagatcacttgaggcttaggagtgtaaagtcccattgaaaccagattgccgtagttctccaacatcacatctctgtataagtccctctgaacagggtccaggcagtcccactcctcctgagagaagtctatggacacatcactgaacatcactgatccctcagccatggcttctagtattgcagatggttagtcttccttgaggccgttctcctgtaatcccagctactcaggaggctgaggcaagagaatcgcttgaacccggaaagcagaggctgcagtgagctgagatcatgccactgcactccagcttgggcaacagagtgagactccgtcttgtatttggtttggtcaacagccattcttcctctgggtaactctcttgacgagagcagagctgaagaagaaaggaatgatgagatgccaggcctttcttgtggcccagactgagcagatcagaggtcattttggatctacagctactatatgcccgacacactcatacatgcccaacactccagaccagcctggtcagtcccttcaaactcccatgcacgtacctgcgggccccagccgagcctgcaagacccaggccgctcaccgcgcacttcccctaccctt

SEQ ID NO: 15620 - RNA, 3458 nt, Homo sapiens
  source 1..3458: mol_type = other RNA
gctgggattacaggcatgagccactgtgcccagccgaggtcagcttttatagctgcaaaaatttagtggcaaccataatgggaatagtcattttaaagtcattaaatatgtcatgaaaataataaaaatctatatttactgaaatggcactcatgaaatctttggcatgataaaagcagttaagggtacagcatgcatatcataattacactttcttaaaaaagcaaagtatagcacgattttctctaccaaattgagagcagccatctataagtatgattacaattaattttggctttttagtttgtaattttttgctttgtgattttggcttaacaattaaaaatgtacatttgtaaaataaaaagaccggccgcagtggctcacgcctgtaatcccagcactttcggaggccgaggcgggtggatcacctgaagtcgggagattgagaccatcctggctaacatggtgaaaccccgtctctactaaaaatacaaaaaattagccgggtgttgtggcacatgcctgtaatcccaactactcaaaaggctgaggcagaagaaccacttgaacctgggaggcgaaggttgtgacgagccgagattgcaccattgcactccagcctaggcaacaagagcgaaactccgtctcaacaaaaaataaagccaggtgcaatcgctcatgcctgtaatcccagcactttgggaggctgaggcaggtggatcacctgaggtcaggagttcaagactatcctgaccaacatggagaaaccctgtctctactaaaaatagaaaattagcagggtgtggtggcacacgcctgtgatcccagctactcaggagtctgaggcaggagaattgcttgaagccgggaggtggaggttgcagcgagccgagattgcgccactgcactccagcctgggcaacagagtgaaactccgtctcaaaaaacatataataataataataaaataaaacaaaaagactaacactaacttcaaaaacaaagttaaacctccacaaggaatttaaaaatattaaaggtcacacaattcaaacagtgtgatactggtgcaaacacaaatacacagatcagaaaagatagctctaaaaacacaagcaaatataaacatgagtataatgtgtcaccaagaaagtagaacaaaacaatgaatgaaagaattatagaacagctggcatcggtatatgactgggggagagagggaatgtcactttagactccgaatttataacctggaatgaaatacatttggatacaaaatttaaatacaaagttttaaaaaaaactacggaagagggtaactattagacatgatttttggtttaaaatatgaggaaggtgacaggggctttaatttttattatttattagtatgaattccctgatgacgaatgagatccgagccactactaaaagccttcccacattccttacagttatagggcttttcaccagtgtgaattctcagatgtcgagtaaggtttgagcatttattaaaggcctttccacattcattacattcatatggtttttcatctgtatgaattctctgatgctggaaaagttgtgagttctgagtaaaggccttcccacattcaagacattcaaagggtttctcaccagcgtgaattctctgatgttgacgaagctgtgagctctgagtaaaagcctttccacattccttacaatcatagggtttctcaccagtgtgaattctctgatgattagtaagtgctgagccactactaaaggctttgccacattccttgcactcatagggtttctcaccagtatgaattctctgatgttgaacaagctttgagctctgggtaaaggctttgccacattccttacattcatagggtttctcacctgtatgaattcgtgcatgctgaaaaagttgtgagctcttagtaaaggctttcccacatactttacattcataaggtttttcaccagtgtgaattcgctgatggtcaataagatttgagcaataactaaaggccttcccacattccttacattcatagggtttcttaccggtatggattctctgatgttgagaaaggtatgagctacaactgaaggcctttccacattccttacattcaaagggtttttcgccagtatgaattttcagatgccgagtaacatgtgaaccacaactaaagaatttcccacactctttacattcataagatttttcaccaatatgaattctctgatgttgaataaattgtgagttctgactaaaggcctttccacatttcttacattcatagggtctgtcttcattattaattatttgatggagagtaaggaatgtctgttgaataaatgtgggcatgtattcaggagtgaatatttcttgactaaaatgcccatttggatatcccagttgttttgcaaggtggcttctatattccaaaacatctccaaaactggagtactcaaggccatgctttgtaagtcccattatctccctctggcataattctatttcataaacttccttctttagagataataacttggtttcacacatcgattccagatctgaacacaggcctcttgtaagctctctgccaaccatccagggctctttcccttgttccaataaggagatcacttgaggcttaggagtgtaaagtcccattgaaaccagattgccgtagttctccaacatcacatctctgtataagtccctctgaacagggtccaggcagtcccactcctcctgagagaagtctatggacacatcactgaacatcactgatccctcagccatggcttctagtattgcagatggttagtcttccttgaggccgttctcctgtaatcccagctactcaggaggctgaggcaagagaatcgcttgaacccggaaagcagaggctgcagtgagctgagatcatgccactgcactccagcttgggcaacagagtgagactccgtcttgtatttggtttggtcaacagccattcttcctctgggtaactctcttgacgagagcagagctgaagaagaaaggaatgatgagatgccaggcctttcttgtggcccagactgagcagatcagaggtcattttggatctacagctactatctgaggtggggaggtcgagaccagcctgaccaacacggagaaaccccgtctctactgaaaatacaaaattagcagggcgtggtgacacacgcctgtaatcccagctactaggaaggctgaggcaggagaattgcttgaaccggggaggcggaggttgcggtgagccgagattgcgccattgcactccagcctgggcaacaacagcgaaactccgcatgcccaacactccagaccagcctggtcagtcccttcaaactcccatgcacgtacctgcgggccccagccgagcctgcaagacccaggccgctcaccgcgcacttcccctaccctt

SEQ ID NO: 15621 - RNA, 3454 nt, Homo sapiens
  source 1..3454: mol_type = other RNA
gctgggattacaggcatgagccactgtgcccagccgaggtcagcttttatagctgcaaaaatttagtggcaaccataatgggaatagtcattttaaagtcattaaatatgtcatgaaaataataaaaatctatatttactgaaatggcactcatgaaatctttggcatgataaaagcagttaagggtacagcatgcatatcataattacactttcttaaaaaagcaaagtatagcacgattttctctaccaaattgagagcagccatctataagtatgattacaattaattttggctttttagtttgtaattttttgctttgtgattttggcttaacaattaaaaatgtacatttgtaaaataaaaagaccggccgcagtggctcacgcctgtaatcccagcactttcggaggccgaggcgggtggatcacctgaagtcgggagattgagaccatcctggctaacatggtgaaaccccgtctctactaaaaatacaaaaaattagccgggtgttgtggcacatgcctgtaatcccaactactcaaaaggctgaggcagaagaaccacttgaacctgggaggcgaaggttgtgacgagccgagattgcaccattgcactccagcctaggcaacaagagcgaaactccgtctcaacaaaaaataaagccaggtgcaatcgctcatgcctgtaatcccagcactttgggaggctgaggcaggtggatcacctgaggtcaggagttcaagactatcctgaccaacatggagaaaccctgtctctactaaaaatagaaaattagcagggtgtggtggcacacgcctgtgatcccagctactcaggagtctgaggcaggagaattgcttgaagccgggaggtggaggttgcagcgagccgagattgcgccactgcactccagcctgggcaacagagtgaaactccgtctcaaaaaacatataataataataataaaataaaacaaaaagactaacactaacttcaaaaacaaagttaaacctccacaaggaatttaaaaatattaaaggtcacacaattcaaacagtgtgatactggtgcaaacacaaatacacagatcagaaaagatagctctaaaaacacaagcaaatataaacatgagtataatgtgtcaccaagaaagtagaacaaaacaatgaatgaaagaattatagaacagctggcatcggtatatgactgggggagagagggaatgtcactttagactccgaatttataacctggaatgaaatacatttggatacaaaatttaaatacaaagttttaaaaaaaactacggaagagggtaactattagacatgatttttggtttaaaatatgaggaaggtgacaggggctttaatttttattatttattagtatgaattccctgatgacgaatgagatccgagccactactaaaagccttcccacattccttacagttatagggcttttcaccagtgtgaattctcagatgtcgagtaaggtttgagcatttattaaaggcctttccacattcattacattcatatggtttttcatctgtatgaattctctgatgctggaaaagttgtgagttctgagtaaaggccttcccacattcaagacattcaaagggtttctcaccagcgtgaattctctgatgttgacgaagctgtgagctctgagtaaaagcctttccacattccttacaatcatagggtttctcaccagtgtgaattctctgatgattagtaagtgctgagccactactaaaggctttgccacattccttgcactcatagggtttctcaccagtatgaattctctgatgttgaacaagctttgagctctgggtaaaggctttgccacattccttacattcatagggtttctcacctgtatgaattcgtgcatgctgaaaaagttgtgagctcttagtaaaggctttcccacatactttacattcataaggtttttcaccagtgtgaattcgctgatggtcaataagatttgagcaataactaaaggccttcccacattccttacattcatagggtttcttaccggtatggattctctgatgttgagaaaggtatgagctacaactgaaggcctttccacattccttacattcaaagggtttttcgccagtatgaattttcagatgccgagtaacatgtgaaccacaactaaagaatttcccacactctttacattcataagatttttcaccaatatgaattctctgatgttgaataaattgtgagttctgactaaaggcctttccacatttcttacattcatagggtctgtcttcattattaattatttgatggagagtaaggaatgtctgttgaataaatgtgggcatgtattcaggagtgaatatttcttgactaaaatgcccatttggatatcccagttgttttgcaaggtggcttctatattccaaaacatctccaaaactggagtactcaaggccatgctttgtaagtcccattatctccctctggcataattctatttcataaacttccttctttagagataataacttggtttcacacatcgattccagatctgaacacaggcctcttgtaagctctctgccaaccatccagggctctttcccttgttccaataaggagatcacttgaggcttaggagtgtaaagtcccattgaaaccagattgccgtagttctccaacatcacatctctgtataagtccctctgaacagggtccaggcagtcccactcctcctgagagaagtctatggacacatcactgaacatcactgatccctcagccatggcttctagtattgcagatggttagtcttccttgaggccgttctcctgtaatcccagctactcaggaggctgaggcaagagaatcgcttgaacccggaaagcagaggctgcagtgagctgagatcatgccactgcactccagcttgggcaacagagtgagactccgtcttgtatttggtttggtcaacagccattcttcctctgggtaactctcttgacgagagcagagctgaagaagaaaggaatgatgagatgccaggcctttcttgtggcccagactgagcagatcagaggtcattttggatctacagctactatctgaggtggggaggtcgagaccagcctgaccaacacggagaaaccccgtctctactgaaaatacaaaattagcagggcgtggtgacacacgcctgtaatcccagctactaggaaggctgaggcaggagaattgcttgaaccggggaggcggaggttgcggtgagccgagattgcgccattgcactccagcctgggcaacaacagcgaaactccgcccaacactccagaccagcctggtcagtcccttcaaactcccatgcacgtacctgcgggccccagccgagcctgcaagacccaggccgctcaccgcgcacttcccctaccctt

SEQ ID NO: 15622 - RNA, 4404 nt, Homo sapiens
  source 1..4404: mol_type = other RNA
gctgggattacaggcatgagccactgtgcccagccgaggtcagcttttatagctgcaaaaatttagtggcaaccataatgggaatagtcattttaaagtcattaaatatgtcatgaaaataataaaaatctatatttactgaaatggcactcatgaaatctttggcatgataaaagcagttaagggtacagcatgcatatcataattacactttcttaaaaaagcaaagtatagcacgattttctctaccaaattgagagcagccatctataagtatgattacaattaattttggctttttagtttgtaattttttgctttgtgattttggcttaacaattaaaaatgtacatttgtaaaataaaaagaccggccgcagtggctcacgcctgtaatcccagcactttcggaggccgaggcgggtggatcacctgaagtcgggagattgagaccatcctggctaacatggtgaaaccccgtctctactaaaaatacaaaaaattagccgggtgttgtggcacatgcctgtaatcccaactactcaaaaggctgaggcagaagaaccacttgaacctgggaggcgaaggttgtgacgagccgagattgcaccattgcactccagcctaggcaacaagagcgaaactccgtctcaacaaaaaataaagccaggtgcaatcgctcatgcctgtaatcccagcactttgggaggctgaggcaggtggatcacctgaggtcaggagttcaagactatcctgaccaacatggagaaaccctgtctctactaaaaatagaaaattagcagggtgtggtggcacacgcctgtgatcccagctactcaggagtctgaggcaggagaattgcttgaagccgggaggtggaggttgcagcgagccgagattgcgccactgcactccagcctgggcaacagagtgaaactccgtctcaaaaaacatataataataataataaaataaaacaaaaagactaacactaacttcaaaaacaaagttaaacctccacaaggaatttaaaaatattaaaggtcacacaattcaaacagtgtgatactggtgcaaacacaaatacacagatcagaaaagatagctctaaaaacacaagcaaatataaacatgagtataatgtgtcaccaagaaagtagaacaaaacaatgaatgaaagaattatagaacagctggcatcggtatatgactgggggagagagggaatgtcactttagactccgaatttataacctggaatgaaatacatttggatacaaaatttaaatacaaagttttaaaaaaaactacggaagagggtaactattagacatgatttttggtttaaaatatgaggaaggtgacaggggctttaatttttattatttattagtatgaattccctgatgacgaatgagatccgagccactactaaaagccttcccacattccttacagttatagggcttttcaccagtgtgaattctcagatgtcgagtaaggtttgagcatttattaaaggcctttccacattcattacattcatatggtttttcatctgtatgaattctctgatgctggaaaagttgtgagttctgagtaaaggccttcccacattcaagacattcaaagggtttctcaccagcgtgaattctctgatgttgacgaagctgtgagctctgagtaaaagcctttccacattccttacaatcatagggtttctcaccagtgtgaattctctgatgattagtaagtgctgagccactactaaaggctttgccacattccttgcactcatagggtttctcaccagtatgaattctctgatgttgaacaagctttgagctctgggtaaaggctttgccacattccttacattcatagggtttctcacctgtatgaattcgtgcatgctgaaaaagttgtgagctcttagtaaaggctttcccacatactttacattcataaggtttttcaccagtgtgaattcgctgatggtcaataagatttgagcaataactaaaggccttcccacattccttacattcatagggtttcttaccggtatggattctctgatgttgagaaaggtatgagctacaactgaaggcctttccacattccttacattcaaagggtttttcgccagtatgaattttcagatgccgagtaacatgtgaaccacaactaaagaatttcccacactctttacattcataagatttttcaccaatatgaattctctgatgttgaataaattgtgagttctgactaaaggcctttccacatttcttacattcatagggtctgtcttcattattaattatttgatggagagtaaggaatgtctgttgaataaatgtgggcatgtattcaggagtgaatatttcttgactaaaatgcccatttggatatcccagttgttttgcaaggtggcttctatattccaaaacatctccaaaactggagtactcaaggccatgctttgtaagtcccattatctccctctggcataattctatttcataaacttccttctttagagataataacttggtttcacacatcgattccagatctgaacacaggcctcttgtaagctctctgccaaccatccagggctctttcccttgttccaataaggagatcacttgaggcttaggagtgtaaagtcccattgaaaccagattgccgtagttctccaacatcacatctctgtataagtccctctgaacagggtccaggcagtcccactcctcctgagagaagtctatggacacatcactgaacatcactgatccctcagccatggcttctagtattgcagatggttagtcttccttgaggccgttctcctgtaatcccagctactcaggaggctgaggcaagagaatcgcttgaacccggaaagcagaggctgcagtgagctgagatcatgccactgcactccagcttgggcaacagagtgagactccgtcttgtatttggtttggtcaacagccattcttcctctgggtaactctcttgacgagagcagagctgaagaagaaaggaatgatgagatgccaggcctttcttgtggcccagactgagcagatcagaggtcattttggatctacagctactatctgaggtggggaggtcgagaccagcctgaccaacacggagaaaccccgtctctactgaaaatacaaaattagcagggcgtggtgacacacgcctgtaatcccagctactaggaaggctgaggcaggagaattgcttgaaccggggaggcggaggttgcggtgagccgagattgcgccattgcactccagcctgggcaacaacagcgaaactccgccttaaaacaaaacaaaacaaaaacagagaagtgtaggctgtcatgagcattcttggtatcagaggggtgaggtctctcctctcgagaatctgtcctgacctcacagggagagctggagtcacaaagacagtcacaagcaccccctacccaatgctgcagtcacccagccaccatggggacccacatagacctccacaggcacgcctcacccaaacaataacactatatatggtcacacaatcattgtcccacatctaccttgaggataagttacactagcatatttacagacccctcaaacatagcaccattcagaaccagagtgctacagatagtcacaataccacacgcactactgagccacacaaagttacagttcccccctccccaggacccctattgagcactacacacaatcacacattcaaaataacacaatgaccactaggacacacatatcaccccggcacgattacacgcactttccaaccgcagacacagtgctacataaagttacatggtcacactctcacattctcacgttactgggttatttctgggtagtagatttactcagtaaggcatccagtacacttaagtgctgctaacagtcatacaaacacaattacacacacccctcagactaacacacagtcacagcctcatcagattctctccacacaaacaccctccacaaatgtcacgcaaagttacacagccacacacaatcacagtcccaacacgggacacagtcatacctacacatacagccttacattgttacaattacacaactacaacgaggatatacaatcacacccgcgcacacagagaggcacagtcacataaggtcacactcacacacggaagcccacgcctcgcgcccgcctccccaccaccccctctatcagcccgaccaactcatacatgcccgacacactcatacatgcccaacactccagaccagcctggtcagtcccttcaaactcccatgcacgtacctgcgggccccagccgagcctgcaagacccaggccgctcaccgcgcacttcccctaccctt

SEQ ID NO: 15623 - RNA, 3188 nt, Homo sapiens
  source 1..3188: mol_type = other RNA
gctgggattacaggcatgagccactgtgcccagccgaggtcagcttttatagctgcaaaaatttagtggcaaccataatgggaatagtcattttaaagtcattaaatatgtcatgaaaataataaaaatctatatttactgaaatggcactcatgaaatctttggcatgataaaagcagttaagggtacagcatgcatatcataattacactttcttaaaaaagcaaagtatagcacgattttctctaccaaattgagagcagccatctataagtatgattacaattaattttggctttttagtttgtaattttttgctttgtgattttggcttaacaattaaaaatgtacatttgtaaaataaaaagaccggccgcagtggctcacgcctgtaatcccagcactttcggaggccgaggcgggtggatcacctgaagtcgggagattgagaccatcctggctaacatggtgaaaccccgtctctactaaaaatacaaaaaattagccgggtgttgtggcacatgcctgtaatcccaactactcaaaaggctgaggcagaagaaccacttgaacctgggaggcgaaggttgtgacgagccgagattgcaccattgcactccagcctaggcaacaagagcgaaactccgtctcaacaaaaaataaagccaggtgcaatcgctcatgcctgtaatcccagcactttgggaggctgaggcaggtggatcacctgaggtcaggagttcaagactatcctgaccaacatggagaaaccctgtctctactaaaaatagaaaattagcagggtgtggtggcacacgcctgtgatcccagctactcaggagtctgaggcaggagaattgcttgaagccgggaggtggaggttgcagcgagccgagattgcgccactgcactccagcctgggcaacagagtgaaactccgtctcaaaaaacatataataataataataaaataaaacaaaaagactaacactaacttcaaaaacaaagttaaacctccacaaggaatttaaaaatattaaaggtcacacaattcaaacagtgtgatactggtgcaaacacaaatacacagatcagaaaagatagctctaaaaacacaagcaaatataaacatgagtataatgtgtcaccaagaaagtagaacaaaacaatgaatgaaagaattatagaacagctggcatcggtatatgactgggggagagagggaatgtcactttagactccgaatttataacctggaatgaaatacatttggatacaaaatttaaatacaaagttttaaaaaaaactacggaagagggtaactattagacatgatttttggtttaaaatatgaggaaggtgacaggggctttaatttttattatttattagtatgaattccctgatgacgaatgagatccgagccactactaaaagccttcccacattccttacagttatagggcttttcaccagtgtgaattctcagatgtcgagtaaggtttgagcatttattaaaggcctttccacattcattacattcatatggtttttcatctgtatgaattctctgatgctggaaaagttgtgagttctgagtaaaggccttcccacattcaagacattcaaagggtttctcaccagcgtgaattctctgatgttgacgaagctgtgagctctgagtaaaagcctttccacattccttacaatcatagggtttctcaccagtgtgaattctctgatgattagtaagtgctgagccactactaaaggctttgccacattccttgcactcatagggtttctcaccagtatgaattctctgatgttgaacaagctttgagctctgggtaaaggctttgccacattccttacattcatagggtttctcacctgtatgaattcgtgcatgctgaaaaagttgtgagctcttagtaaaggctttcccacatactttacattcataaggtttttcaccagtgtgaattcgctgatggtcaataagatttgagcaataactaaaggccttcccacattccttacattcatagggtttcttaccggtatggattctctgatgttgagaaaggtatgagctacaactgaaggcctttccacattccttacattcaaagggtttttcgccagtatgaattttcagatgccgagtaacatgtgaaccacaactaaagaatttcccacactctttacattcataagatttttcaccaatatgaattctctgatgttgaataaattgtgagttctgactaaaggcctttccacatttcttacattcatagggtctgtcttcattattaattatttgatggagagtaaggaatgtctgttgaataaatgtgggcatgtattcaggagtgaatatttcttgactaaaatgcccatttggatatcccagttgttttgcaaggtggcttctatattccaaaacatctccaaaactggagtactcaaggccatgctttgtaagtcccattatctccctctggcataattctatttcataaacttccttctttagagataataacttggtttcacacatcgattccagatctgaacacaggcctcttgtaagctctctgccaaccatccagggctctttcccttgttccaataaggagatcacttgaggcttaggagtgtaaagtcccattgaaaccagattgccgtagttctccaacatcacatctctgtataagtccctctgaacagggtccaggcagtcccactcctcctgagagaagtctatggacacatcactgaacatcactgatccctcagccatggcttctagtattgcagatggttagtcttccttgaggccgttctcctgtaatcccagctactcaggaggctgaggcaagagaatcgcttgaacccggaaagcagaggctgcagtgagctgagatcatgccactgcactccagcttgggcaacagagtgagactccgtcttgtatttggtttggtcaacagccattcttcctctgggtaactctcttgacgagagcagagctgaagaagaaaggaatgatgagatgccaggcctttcttgtggcccagactgagcagatcagaggtcattttggatctacagctactatctgcgggccccagccgagcctgcaagacccaggccgctcaccgcgcacttcccctaccctt

SEQ ID NO: 15624 - RNA, 3099 nt, Homo sapiens
  source 1..3099: mol_type = other RNA
gctgggattacaggcatgagccactgtgcccagccgaggtcagcttttatagctgcaaaaatttagtggcaaccataatgggaatagtcattttaaagtcattaaatatgtcatgaaaataataaaaatctatatttactgaaatggcactcatgaaatctttggcatgataaaagcagttaagggtacagcatgcatatcataattacactttcttaaaaaagcaaagtatagcacgattttctctaccaaattgagagcagccatctataagtatgattacaattaattttggctttttagtttgtaattttttgctttgtgattttggcttaacaattaaaaatgtacatttgtaaaataaaaagaccggccgcagtggctcacgcctgtaatcccagcactttcggaggccgaggcgggtggatcacctgaagtcgggagattgagaccatcctggctaacatggtgaaaccccgtctctactaaaaatacaaaaaattagccgggtgttgtggcacatgcctgtaatcccaactactcaaaaggctgaggcagaagaaccacttgaacctgggaggcgaaggttgtgacgagccgagattgcaccattgcactccagcctaggcaacaagagcgaaactccgtctcaacaaaaaataaagccaggtgcaatcgctcatgcctgtaatcccagcactttgggaggctgaggcaggtggatcacctgaggtcaggagttcaagactatcctgaccaacatggagaaaccctgtctctactaaaaatagaaaattagcagggtgtggtggcacacgcctgtgatcccagctactcaggagtctgaggcaggagaattgcttgaagccgggaggtggaggttgcagcgagccgagattgcgccactgcactccagcctgggcaacagagtgaaactccgtctcaaaaaacatataataataataataaaataaaacaaaaagactaacactaacttcaaaaacaaagttaaacctccacaaggaatttaaaaatattaaaggtcacacaattcaaacagtgtgatactggtgcaaacacaaatacacagatcagaaaagatagctctaaaaacacaagcaaatataaacatgagtataatgtgtcaccaagaaagtagaacaaaacaatgaatgaaagaattatagaacagctggcatcggtatatgactgggggagagagggaatgtcactttagactccgaatttataacctggaatgaaatacatttggatacaaaatttaaatacaaagttttaaaaaaaactacggaagagggtaactattagacatgatttttggtttaaaatatgaggaaggtgacaggggctttaatttttattatttattagtatgaattccctgatgacgaatgagatccgagccactactaaaagccttcccacattccttacagttatagggcttttcaccagtgtgaattctcagatgtcgagtaaggtttgagcatttattaaaggcctttccacattcattacattcatatggtttttcatctgtatgaattctctgatgctggaaaagttgtgagttctgagtaaaggccttcccacattcaagacattcaaagggtttctcaccagcgtgaattctctgatgttgacgaagctgtgagctctgagtaaaagcctttccacattccttacaatcatagggtttctcaccagtgtgaattctctgatgattagtaagtgctgagccactactaaaggctttgccacattccttgcactcatagggtttctcaccagtatgaattctctgatgttgaacaagctttgagctctgggtaaaggctttgccacattccttacattcatagggtttctcacctgtatgaattcgtgcatgctgaaaaagttgtgagctcttagtaaaggctttcccacatactttacattcataaggtttttcaccagtgtgaattcgctgatggtcaataagatttgagcaataactaaaggccttcccacattccttacattcatagggtttcttaccggtatggattctctgatgttgagaaaggtatgagctacaactgaaggcctttccacattccttacattcaaagggtttttcgccagtatgaattttcagatgccgagtaacatgtgaaccacaactaaagaatttcccacactctttacattcataagatttttcaccaatatgaattctctgatgttgaataaattgtgagttctgactaaaggcctttccacatttcttacattcatagggtctgtcttcattattaattatttgatggagagtaaggaatgtctgttgaataaatgtgggcatgtattcaggagtgaatatttcttgactaaaatgcccatttggatatcccagttgttttgcaaggtggcttctatattccaaaacatctccaaaactggagtactcaaggccatgctttgtaagtcccattatctccctctggcataattctatttcataaacttccttctttagagataataacttggtttcacacatcgattccagatctgaacacaggcctcttgtaagctctctgccaaccatccagggctctttcccttgttccaataaggagatcacttgaggcttaggagtgtaaagtcccattgaaaccagattgccgtagttctccaacatcacatctctgtataagtccctctgaacagggtccaggcagtcccactcctcctgagagaagtctatggacacatcactgaacatcactgatccctcagccatggcttctagtattgcagatggttagtcttccttgaggccgttctcctgtaatcccagctactcaggaggctgaggcaagagaatcgcttgaacccggaaagcagaggctgcagtgagctgagatcatgccactgcactccagcttgggcaacagagtgagactccgtcttgtatttggtttggtcaacagccattcttcctctgggtaactctcttgacgagagcagagctgcgggccccagccgagcctgcaagacccaggccgctcaccgcgcacttcccctaccctt

SEQ ID NO: 15625 - RNA, 4282 nt, Homo sapiens
  source 1..4282: mol_type = other RNA
gctgggattacaggcatgagccactgtgcccagccgaggtcagcttttatagctgcaaaaatttagtggcaaccataatgggaatagtcattttaaagtcattaaatatgtcatgaaaataataaaaatctatatttactgaaatggcactcatgaaatctttggcatgataaaagcagttaagggtacagcatgcatatcataattacactttcttaaaaaagcaaagtatagcacgattttctctaccaaattgagagcagccatctataagtatgattacaattaattttggctttttagtttgtaattttttgctttgtgattttggcttaacaattaaaaatgtacatttgtaaaataaaaagaccggccgcagtggctcacgcctgtaatcccagcactttcggaggccgaggcgggtggatcacctgaagtcgggagattgagaccatcctggctaacatggtgaaaccccgtctctactaaaaatacaaaaaattagccgggtgttgtggcacatgcctgtaatcccaactactcaaaaggctgaggcagaagaaccacttgaacctgggaggcgaaggttgtgacgagccgagattgcaccattgcactccagcctaggcaacaagagcgaaactccgtctcaacaaaaaataaagccaggtgcaatcgctcatgcctgtaatcccagcactttgggaggctgaggcaggtggatcacctgaggtcaggagttcaagactatcctgaccaacatggagaaaccctgtctctactaaaaatagaaaattagcagggtgtggtggcacacgcctgtgatcccagctactcaggagtctgaggcaggagaattgcttgaagccgggaggtggaggttgcagcgagccgagattgcgccactgcactccagcctgggcaacagagtgaaactccgtctcaaaaaacatataataataataataaaataaaacaaaaagactaacactaacttcaaaaacaaagttaaacctccacaaggaatttaaaaatattaaaggtcacacaattcaaacagtgtgatactggtgcaaacacaaatacacagatcagaaaagatagctctaaaaacacaagcaaatataaacatgagtataatgtgtcaccaagaaagtagaacaaaacaatgaatgaaagaattatagaacagctggcatcggtatatgactgggggagagagggaatgtcactttagactccgaatttataacctggaatgaaatacatttggatacaaaatttaaatacaaagttttaaaaaaaactacggaagagggtaactattagacatgatttttggtttaaaatatgaggaaggtgacaggggctttaatttttattatttattagtatgaattccctgatgacgaatgagatccgagccactactaaaagccttcccacattccttacagttatagggcttttcaccagtgtgaattctcagatgtcgagtaaggtttgagcatttattaaaggcctttccacattcattacattcatatggtttttcatctgtatgaattctctgatgctggaaaagttgtgagttctgagtaaaggccttcccacattcaagacattcaaagggtttctcaccagcgtgaattctctgatgttgacgaagctgtgagctctgagtaaaagcctttccacattccttacaatcatagggtttctcaccagtgtgaattctctgatgattagtaagtgctgagccactactaaaggctttgccacattccttgcactcatagggtttctcaccagtatgaattctctgatgttgaacaagctttgagctctgggtaaaggctttgccacattccttacattcatagggtttctcacctgtatgaattcgtgcatgctgaaaaagttgtgagctcttagtaaaggctttcccacatactttacattcataaggtttttcaccagtgtgaattcgctgatggtcaataagatttgagcaataactaaaggccttcccacattccttacattcatagggtttcttaccggtatggattctctgatgttgagaaaggtatgagctacaactgaaggcctttccacattccttacattcaaagggtttttcgccagtatgaattttcagatgccgagtaacatgtgaaccacaactaaagaatttcccacactctttacattcataagatttttcaccaatatgaattctctgatgttgaataaattgtgagttctgactaaaggcctttccacatttcttacattcatagggtctgtcttcattattaattatttgatggagagtaaggaatgtctgttgaataaatgtgggcatgtattcaggagtgaatatttcttgactaaaatgcccatttggatatcccagttgttttgcaaggtggcttctatattccaaaacatctccaaaactggagtactcaaggccatgctttgtaagtcccattatctccctctggcataattctatttcataaacttccttctttagagataataacttggtttcacacatcgattccagatctgaacacaggcctcttgtaagctctctgccaaccatccagggctctttcccttgttccaataaggagatcacttgaggcttaggagtgtaaagtcccattgaaaccagattgccgtagttctccaacatcacatctctgtataagtccctctgaacagggtccaggcagtcccactcctcctgagagaagtctatggacacatcactgaacatcactgatccctcagccatggcttctagtattgcagatggttagtcttccttgaggccgttctccttgtatttggtttggtcaacagccattcttcctctgggtaactctcttgacgagagcagagctgaagaagaaaggaatgatgagatgccaggcctttcttgtggcccagactgagcagatcagaggtcattttggatctacagctactatctgaggtggggaggtcgagaccagcctgaccaacacggagaaaccccgtctctactgaaaatacaaaattagcagggcgtggtgacacacgcctgtaatcccagctactaggaaggctgaggcaggagaattgcttgaaccggggaggcggaggttgcggtgagccgagattgcgccattgcactccagcctgggcaacaacagcgaaactccgccttaaaacaaaacaaaacaaaaacagagaagtgtaggctgtcatgagcattcttggtatcagaggggtgaggtctctcctctcgagaatctgtcctgacctcacagggagagctggagtcacaaagacagtcacaagcaccccctacccaatgctgcagtcacccagccaccatggggacccacatagacctccacaggcacgcctcacccaaacaataacactatatatggtcacacaatcattgtcccacatctaccttgaggataagttacactagcatatttacagacccctcaaacatagcaccattcagaaccagagtgctacagatagtcacaataccacacgcactactgagccacacaaagttacagttcccccctccccaggacccctattgagcactacacacaatcacacattcaaaataacacaatgaccactaggacacacatatcaccccggcacgattacacgcactttccaaccgcagacacagtgctacataaagttacatggtcacactctcacattctcacgttactgggttatttctgggtagtagatttactcagtaaggcatccagtacacttaagtgctgctaacagtcatacaaacacaattacacacacccctcagactaacacacagtcacagcctcatcagattctctccacacaaacaccctccacaaatgtcacgcaaagttacacagccacacacaatcacagtcccaacacgggacacagtcatacctacacatacagccttacattgttacaattacacaactacaacgaggatatacaatcacacccgcgcacacagagaggcacagtcacataaggtcacactcacacacggaagcccacgcctcgcgcccgcctccccaccaccccctctatcagcccgaccaactcatacatgcccgacacactcatacatgcccaacactccagaccagcctggtcagtcccttcaaactcccatgcacgtacctgcgggccccagccgagcctgcaagacccaggccgctcaccgcgcacttcccctaccctt

SEQ ID NO: 15626 - RNA, 2977 nt, Homo sapiens
  source 1..2977: mol_type = other RNA
gctgggattacaggcatgagccactgtgcccagccgaggtcagcttttatagctgcaaaaatttagtggcaaccataatgggaatagtcattttaaagtcattaaatatgtcatgaaaataataaaaatctatatttactgaaatggcactcatgaaatctttggcatgataaaagcagttaagggtacagcatgcatatcataattacactttcttaaaaaagcaaagtatagcacgattttctctaccaaattgagagcagccatctataagtatgattacaattaattttggctttttagtttgtaattttttgctttgtgattttggcttaacaattaaaaatgtacatttgtaaaataaaaagaccggccgcagtggctcacgcctgtaatcccagcactttcggaggccgaggcgggtggatcacctgaagtcgggagattgagaccatcctggctaacatggtgaaaccccgtctctactaaaaatacaaaaaattagccgggtgttgtggcacatgcctgtaatcccaactactcaaaaggctgaggcagaagaaccacttgaacctgggaggcgaaggttgtgacgagccgagattgcaccattgcactccagcctaggcaacaagagcgaaactccgtctcaacaaaaaataaagccaggtgcaatcgctcatgcctgtaatcccagcactttgggaggctgaggcaggtggatcacctgaggtcaggagttcaagactatcctgaccaacatggagaaaccctgtctctactaaaaatagaaaattagcagggtgtggtggcacacgcctgtgatcccagctactcaggagtctgaggcaggagaattgcttgaagccgggaggtggaggttgcagcgagccgagattgcgccactgcactccagcctgggcaacagagtgaaactccgtctcaaaaaacatataataataataataaaataaaacaaaaagactaacactaacttcaaaaacaaagttaaacctccacaaggaatttaaaaatattaaaggtcacacaattcaaacagtgtgatactggtgcaaacacaaatacacagatcagaaaagatagctctaaaaacacaagcaaatataaacatgagtataatgtgtcaccaagaaagtagaacaaaacaatgaatgaaagaattatagaacagctggcatcggtatatgactgggggagagagggaatgtcactttagactccgaatttataacctggaatgaaatacatttggatacaaaatttaaatacaaagttttaaaaaaaactacggaagagggtaactattagacatgatttttggtttaaaatatgaggaaggtgacaggggctttaatttttattatttattagtatgaattccctgatgacgaatgagatccgagccactactaaaagccttcccacattccttacagttatagggcttttcaccagtgtgaattctcagatgtcgagtaaggtttgagcatttattaaaggcctttccacattcattacattcatatggtttttcatctgtatgaattctctgatgctggaaaagttgtgagttctgagtaaaggccttcccacattcaagacattcaaagggtttctcaccagcgtgaattctctgatgttgacgaagctgtgagctctgagtaaaagcctttccacattccttacaatcatagggtttctcaccagtgtgaattctctgatgattagtaagtgctgagccactactaaaggctttgccacattccttgcactcatagggtttctcaccagtatgaattctctgatgttgaacaagctttgagctctgggtaaaggctttgccacattccttacattcatagggtttctcacctgtatgaattcgtgcatgctgaaaaagttgtgagctcttagtaaaggctttcccacatactttacattcataaggtttttcaccagtgtgaattcgctgatggtcaataagatttgagcaataactaaaggccttcccacattccttacattcatagggtttcttaccggtatggattctctgatgttgagaaaggtatgagctacaactgaaggcctttccacattccttacattcaaagggtttttcgccagtatgaattttcagatgccgagtaacatgtgaaccacaactaaagaatttcccacactctttacattcataagatttttcaccaatatgaattctctgatgttgaataaattgtgagttctgactaaaggcctttccacatttcttacattcatagggtctgtcttcattattaattatttgatggagagtaaggaatgtctgttgaataaatgtgggcatgtattcaggagtgaatatttcttgactaaaatgcccatttggatatcccagttgttttgcaaggtggcttctatattccaaaacatctccaaaactggagtactcaaggccatgctttgtaagtcccattatctccctctggcataattctatttcataaacttccttctttagagataataacttggtttcacacatcgattccagatctgaacacaggcctcttgtaagctctctgccaaccatccagggctctttcccttgttccaataaggagatcacttgaggcttaggagtgtaaagtcccattgaaaccagattgccgtagttctccaacatcacatctctgtataagtccctctgaacagggtccaggcagtcccactcctcctgagagaagtctatggacacatcactgaacatcactgatccctcagccatggcttctagtattgcagatggttagtcttccttgaggccgttctccttgtatttggtttggtcaacagccattcttcctctgggtaactctcttgacgagagcagagctgcgggccccagccgagcctgcaagacccaggccgctcaccgcgcacttcccctaccctt

SEQ ID NO: 15627 - RNA, 13676 nt, Homo sapiens
  source 1..13676: mol_type = other RNA
gctgggattacaggcatgagccactgtgcccagcctaaagcgtaataaactttcactgttgctctgaaacttgcctcggtccctccttctgccttatgcccctcagtcaaattctttcttctgaggaggaaagaattgaggttgctgcagatttaccaccagtaacttggataccgtccaccagtaacaacttccgttaagatggcaatacacctcaaatttatttttattttgagacagggtctcactctgttccccaggctggagtacagtggcacaatctcagctcactgaaacctccacctcccgggctcaagtgatcctcccacctcagccttccgagtagctggtactacaggcgcatgctaccatacccagctaatttttgtatttttagtagagacagggttttgccgtgttgcccaaggtggcctcaaattccttggctcaagcgatccaccatcctcagcctcccaaagtcctgggattacaggcatgagccactgcgcccagccaaacttatctttgtatgtttgttataggcaaaagtaccccaaggttaaggctcagcccaagaggtcaagtgggttcaggaaagaattcaagagcatgctgacagaataaagtgaaagcaagttcattaagaaagtaaaggaataaaagaatggctaccccataggaagagtagccctgatgggctgctgactggctatatttatggttgcttcttgactatacgctaaacaagaggtggcttattcatgagttttccaggaaagaagtggggaggtctggaccttttagaccatacagggtaacttctgaaagttgctatggcagttgtaaactatcatggtgctgtagaagtttcttttagcgtgctaatgtattataattaccatagaatgggcagcaaaggtaaccagaggtctcttctgtcaccatcatggttttggctggtttgggttggcctttctaccacatcctgtcttatcagcagggtcttacagggtcttgtggtcttgggaaaccagtcctgccaaactcctctcattcagtgtaatcactatcaaaattccagaggccctttttacataaatttgcaagtgaatcctaacagttatatgaaaatttagggaaaggtaaacccaatacagccctaacaattttgaaaaagaacaggccagttgcagtggctcacccctcagcactttgggaggtggaggtgggaggattgtttgaggccaggagtttgagaccagcctgggcaacatagcaaggcctcatctctacaaaagaaaaaagaagaacaacaacaacaacaaagttagaggactacatttctggattccaaaacttactacgaagttacaataatcaagacagtgtggtactaccataagatagagcaacagaattgagtccagaaataaacccttatagttagttgatttgtgataagtataaaataattctatagggaaaaaatagtattttcaataagtaatgctaagacaagtgaacatttatgtgcaaaagaatgaggctggatgcttatctcgcactgcatacacaaaaataactcaaaatgggtcaaagagctaaaatcataaaactttagaagaaaacataggggtaacacctcataggcaattgatttagacaatggttttttaggtatgacaccaaaagcataagcaataacataaaaaacagaaatcaagtgaacttcatcaaaatttaaaacttgtactgtatagtatccagaaagtgagaagacaatccatggaatgggagaatatattcacaaagattgtacctgataagaaactagtatccagaatattaaaaagaatgcttacaactcaacaataaaaagacaacccaccgggtgtggtggctcacgcctgtaatcctagcattttgggaggccgaggcaggcagatcacctgagttcaggagttcaagaccagcctggccaacatggcgaaaccctgtctctactaaaaatacaaaaattagccaggcgtgatggtgggtgcctgtaatcccagttactagggaggccgaggcaggagagtcgcttgaactcaggaggtggaggttgcagtgagccgagattgcaccactgcactccaacctgggcgacagagtgagattccatctcagaaaaataaaataaaataacgcagttttaaaatgagaaaggacttgaggccaggcacagtagctaatgtctgtaatgccagcactttgggaagccaaggcagtcagatcacctgaggccaggagttcgagaccagcctggccaacatggtgaaaccctgtctttactaaaaatacaaaaattggctgggcgcggtggctcacgcctgtaatcccagcactttgggaggccaaggcaggcggatcacgaggtcaggagatagagaccatcctggctaacacggtgaaaccctgtctctactaaaaatacaaaaaattagccgggcgtggtggagggcggctgtagtcccagatacttgggaggctgaggcaggagaatggcatgaacccaggaggcggagcttgcagtgagctgagattgcaccactgcactccagcctgggccacagagcgagactccgtctcaaaaaacaatacaaaaattagttgggcatggtggcgagctcctgtaaacccagctactcccaactactagggaggctgaggcaggagaatggcttgaacccagaaggcagaggttacagtgaatcaagataacgccactgcactccaccctgggcgacagagtgagactccgtctcaaaaacaaaaaaataaaaaaaacctcatacactgctggtgggaatataaaatgatgctactactttgaaaagcagtttggcagttcctcaaaaggctaaacatagagttactatatgatgagcactctcacttctaaggtatatgcccagaagaactgaaaacatatatccatataaaaattcatatacgaatattcatagcagcatcatccataatagcaaaaaagtggaaacagtctaaatttcgatcaactgatgaataaactaaatgcggtatatccacacaatagggtattattcagccataaaatgtaatgaagcactggtacactctatagcatagatgaaccttgaaacatgctaagtgaaggaagtcagacacgaaaggccacatgtttatttttataaaatatctagaacaggcaaatcatagagacagaaaatggattattgtttctagaggctgggggaagaggaggattagagtggcagctcactggtatggagtttctaggtagatggaaatgttctggaattagatagtggtgatgattgcacaactctgtaaatatactaaaatccactgcatcatttactttaaaggggcaaattttatggcttgtgaattacatttcaataaaaagaagatgaggaaacctaggatatgtcacaatcccatgccacaaactacttacacttccaatataaaaactatatcaacaatagtttacatcacgttcattgcttgctaaagtaaggtcatgaatgtatcaaaatattttataaaagttaaaatttaggagatccatcatttctcttttcaatccatcactgattcattcaatatatatttatgtgtatgccaggctcttcatcaggtaaagtgtttaggagagatataaagataaaactgatgagaattctgcacttgagctacagcatactttccaagaattacagcatgagatataaaatgaaaagaaggcttggaggagattcacacgaaatagtactgttcaggagagggggcgataattccaatggaagagataactgacttcatggaggatagaaggagatggtatttgaactgcccttgaagtatggttatattttggggatgtggagatgtggggtagggtgatatgctggggttccagatggtccagaaatatacaatcaccagaaccaaagatccagaggtaggagatatgagctgttcaatttggctgagctaacagtgtttggagtgggatcttgaagaagctgaaaatgaagataccaactagacagtcagagaaagacttccaatgtttgactgaactgcaattttattgtgtatgcattgaagaatctttttttttttttttgtattctctaaagatttttaaaatattttaagttctggatacaagtgcaggatgtgcgggtttgttacataggtaaacgtgtcccatggtggtttgctgcacctatcaacctatcacctaggtattaagccccacatgcattagctagttatcctgatgctctccccgctacggcccctgcatcaggccccagtgtgtgttgatctcatccctgtgtccgtgtgttctcattgttcagcttccgcttacaagtgagaacatgtggtgtttggtttcctgctcctctgttagtttgctgaggataatggcttccagcttcatccatgtccctgcaaaggacatgatctcattccttttttaaaaaaaaaaacaaaattatttccataggtgtttggggaacaggtggtatctggttacatgcgtaagtaattaagtggttacttgtgagattctggtgcacccatcacctgagcagtatacactgaacccaatttgtattcttttatccttcacccccctcccaccctttcccctaagtccccaaagtccattgtatccttcttatgcctttgcatcctcatagcttatctcccacttatgagtgagaacatacaatgtttggttttccattcctcagttacttcctttagagtaatagtctccaggttgctgtgaatgtcattaattcattcctttttatggctgagtagtgtttaggtgaggttatttgtaagtaattaatattgagtaaataagattcatccatagtggcaaagccacataacttctaagtatcttaaactatatctaaatggtaccaaaacatgcagtcaattctaaaagctcagctaatgatatttcataatataggaaaatattcacaacatatttttgtgtaaaaaaaagcagacttcaaaatggaatatgcattatgattccaatcatgtaaaagctatacatgaacacatacaaagattaacagatataaacaaatggaagaatgaatggagagatagatgatagacagattgagtggtggtggagaataacagatttaaaaagaaattgtgcctttctatattttcaaaaccatttaaataagtattacctttggagttagaaaatgatatgtattttaaatccataattcaactacttatctatatgatgtcaaactggattaggctgaattatcagcaagtgaataaaacagttccttcatccatggagaaacatccatttatgacattcttggaattcctcttgttagaattctttatgaatttaaaatagaaacatggccagactcaagatttcaatacaaacattactttttcacgttcagtaataaccaattaaaagaattaatgaaaaatctgattcactgtatcaccaaaagctgtaatggctgcactgcacagtattccatggtgtatatgtaccacattttctttatccagtctatctttgatgggcatttgctattgtgtctttgctattgtgaagagtgctgcaatgaacaaaaatgtgcatgtatctttataataaaatggtttatattcctttgggtatatacccagtaatgggattgctgggacaaatagtatttctagttctagatctttgaggaatagccacacacacttccacaacggttgaactaatttacattcccaccaacaatgtaaaagtgttcctacttctccacagcctcgccagcatctgttgttttttgactttttaataatcaccattctgaccggcatgagatggtatctcattgtggttctcctttgcatttctctaatgatcagtaaggttgagcttttttttatatgtttgttggccacataaatgtcttcttttgagaagtgtctgttcatgtcctttgtccactttttgatggggttgtttttttccttgtaaatttgttttaagttccttgtaggttctggatattagacctttgtcagatggatagattgcaaaaatgttctcccattctgtaggttgcctgttcactctaatgatagtttcttttgctgtgcaggagctctttagtttaattagatcccatttgtaatttttgcttttgttgcaattgcttttgatgtttttgtcatgaaacctttgcttgtgcctatgtcttgaatggtattaaatagattttcttctagggtttttatagttttaggttttacattaagtctttaatcttgagttaatttttgtataaggtgtaaggaaggggtcagtttcaattttctgcatatggctagccagttttcccagcaccatttattaaatagggaatcttttccccattgcttgtttttgtcaggtttgtcgatgatcagatggctgtagatgtgtggtcttctttctctggtctctattctgttccattggtctatgtgtctgtttttgtaccagtaccatgccattttggctactgtagccttgcagtatactttgaagttgggtagtgtgatgcttccagctttgttctttttgcttattgttgtcttggttatacgggctcttttttggttccatttgaattttaaagtagtttttttctaattctgtgaagaatgtcaatagtagtttaatgggaatagcaatgaacctataaattactttgggtagtatggccattttcatgatattgattcttcctatccacgagaatggaatgttttttcatttgtgtcctctcttatttccttgagcagtggtttgtagttctccttgaagagatccttcacatcttattagctgtattcctaggtattttattctctttctagcaactgtgaatgggagttcattcatgatttggctctctgcttgtgtattgttggtgtatagaatgcttgtgatttctgcacattgattttgtatcctgagactttgctgaagttgcttatcagcttaaggaacttttgggtggagataatggggttttctagatatagtatcatgtcatctgcaaacacagttttacttcctcttttcctatttgaataccccttatttgtttctcttgcctgattttcttggccagaacttccaatactatgttaaataggagtggtgagacggcatccctgtcttgtgccagttttcaaggggaatgcttccagcttttgcccattcagtatgataatggctgtgggtttgtcataaatggttattattttgagatattttccatcaatacctagtttattgagagtttttaacatgaagcaacgttgaattttattgaaggccttttctgtatctattgagataatcatgtggtttttgtctttagttctgtttatgtgatgaattatgtttcttgatttgcgtatgttgaaccagccttgcatcccagggatgaagccaacattccaaacattttatttattatttatttatttatttatttttgagacagagtctcgcactgtcgcccaggctggagtgcagtggcaagatctcagctcgctgcaagctccacctcccaggttcatgccgttctcttgcctcggcctcccaaatagcagggactacaggcgaccgccacaacgcctggctaattttttgtatttttagtagagacggggttttacatgttagccaggatggtcttgatctcctgacctcgtgatccgcccgccttggcctcccaaagggctgggattataggcgtgagccaccgcacccggcctccaaacattttaatctcataacaatgcatcacttgggttaactaggttgagataaatataaactgtcaattttttttcccctcacataaaagtccagaggtaggtaattagggctgacacagtgattccagtgattctgctccttcgtgccctcatccaacaaggcttcttgctgctcactacccagctacccctacgtgtggcccgtatcttcatggttcaagatggcagctagagctgctaggtagttaagatctctctcacacactttccttctgtcataattaacacagggttttagctcatgaggccaagcatacacattacttcccactggcacccctatgtaatattaaatgcaaagataccctcaggagtcctgtgctcaaaacaagtacaaaataactttttgttgttgtttgtggtgctggtggttttatttatttattttttctgaaacagggtctcactctgtctcccatgctgaagtgcagtggtgtgatcacagctcatcacaaccttgacctctctgggctcaggggatccactcacttcagcctcccaagtagctgggactacaggaacacgccaccacgctcagctaaattttgtctttttttgtagagatggagtcttgctatgttgcccaggctggtctcaaactcctgggctcaagtgatcagtccacctcagcctcccaaagtactcagattataggtatgagccaccatggcatcaaaataacttggaaagtaggaataattgcttgttgttcctgaaaactgtctcttcgacacttttcagactctgttacatgatcatgacaaaatatacacaaatagacatacagatacacatcagttaaaacctcaagaaatagaaaaataaataaatcataaaatatttaaaaagtggtattctgacacactgcccagaggtacccctgttcagcaattttaaaaaattttaaaaatagccctctccccctccctctcttctccctctccccacggtctccctctgatgccgagccgaagctggactgtactgctgccatctcggctcactgcagcctccctgcctgattctcccgcctcggcctgccgcgtgcctgccattgcgggcgccgccacgcctgactggttttcgtatttttttggtggagacagggtttcactgtgttggccgggctggtctccagctcctgactgcgagtgatctgccagcctcggcctcccgaggtgccgggattgcgggcagagtctcgtccactcagtgctcaatgttgcccaggctggagtgcagtggtgtgatctcagctggctacggcctccgcctcccagccgcctgccttggccccccagggtgccgagattacagcttctgcccggccgccaccccgtctgggatgaagtgaggagcgtctctgcccggccgcccatcgtctgagatgtggggagcgcctctgccccgcccccccgtctgggatgtgaggagcttctctgcccggccaccccgtctgagaagtgaggagcccctccgcccgcagctgccccgtctgagaagtgaggagcccctccgcccgacagccaccctgtctgggaagtgaggagcgtctccgcccagcagccaccccgtctgagaagtgaggagcccctccgcctggcagccgccccgtccgggagggaggcgtgggggtcagcccccgcccggccagccgccccgtcggggagggaggtggggggtcagcccccgcccggccagctatcccgtccgggagggaggtggggggcgcgtccgcctggccgccccatctgggaagtgaggagcccctctgcccagccgccaccccgtctgggaggtgtacccaacagctcattgagaacaggccatgatgacgatggcggttttgtggaatagaaaagggggaaaggtggggaaaagatagagaaatcagattgttgctgtgtctgtgtagaaagaagtagacatgggagacttcattttgttctgtactaagaaaaattcttctgccttaggatgctgttgatctatgaccttacccccaaccctgtgctctctgaaacatgtgctgtgtccactcagggttaaatggattaagggcagtgcaagatgtgctttgttaaacagatgcttgaaggcagcatgctccttaagagtcatcaccactccctaatctcaagtacccagggacacaaacactgcggaaggccgcagggtcctctgcctaggaaaaccagagacctttgttcacttgtttatctgctgaccttccctccactattgtcctgtgaccctgccaaatcaccctctgtgagaaacacccaagaatgatcaattaaaaaaaaaaaatttaaaaataataataggccaggtgcagtggctcacacctgtaatcccagcactttgggaggccgaggctggtgaatcacctgaggtcaggagttcaagaccacgctggccaacatggtggaaaccctgtctccactaaaaatacaaaaattagccgggtgtggtggcaggagcctgtaatcccagctactcgggaggctgaggcaggagaatcgcttgaacccagaaggcagaggttgcaatgagccaagatgatgccactgcactccagcctgggcagcagaatgaaactctgtctcaataataataataataataataataataataataataataataataagcaactctaatgatatttcaaacaatggtccccttttaggtcacactatcaaatcagagaaagatatacttgactagctgtaaaatgcaatttgaggtctaggtgaatgaacaagtaacctctaaatcataaggctattgttacaaactgaatgtttgtattccccccagaattcaaaggggagacagtatccccaaagtgacagtatcagaaggtggggcctttgggaggtaattaggtgatgagggtagagccctcatgaatggaatttgtgcccttaaagatatacttgagagtttgcatcctctttttctgccatgtgagaacatcaaaagactgacatctggtaagatctggaagcatgccttaccagacaccagatatgctaccacttagatgttggatttcccagcctccggaactgtgagaaataactgctgtttaagtcacctggtctatggtaatttggtatagttgcccaaatggactgtgatggttaatactgagtatcaacttgattgaatagaaggatgcaaagtgttcccgggtacatctgtgagggtgctgccaaaggagatttaacatttgagtcagtggactgggaaaggcagaccatcctcaatctgggtgggcaccatctaatcagctgccagcactgccagaataaaagcaggcaaaacatggaaagactagactggtgtagtcttctggcctccatctttctctcatgctgaatgcttcctgccctcaaacattggactccaagttcttcagctttgggacttgaattggcttccttgcttgcagatgacctattgtgggacctaaccctgtgatcatgtgagtcaatactccttaataaactcccctttttatatacatgtatcctattagttctgtccctctagagaaacatgactaatacattgagtaagatagttcctgtcctttttttttttttttaaagagatgggatcttgctatattgcccaggttggtatgcagtggctattcgtaggcacaatcacagcatgctatgaccctgaactcctgggttcaaaagatcctcccacctcagcctcccaagtaactgggaatacaggtacccacacccacacccagctaatttttgtatttttactagggacagcgtttaccatgttggccaggctggtctcgaactcctgacctgaagtgatctgccctccttggcctcccaaagtgctgggattacaggtgtgagccactacgcccagccttttggtttcttatgtgtaggagaggataagtttctttctcagagtgtgctgcagccagacataatatttctccttggcagaaactctgctgttccaatcatacatgtagccattgagttcaatgtgaagatccaggagtgggcgttttctttcttgtctcagtttctgggagaggcactgcaggtacagggatggtgagctgtgagactgctccagcagggacatgtccgcagtacacaggctccagaagaagtcagcttctcggtgaactgtgcacagccctcgcttctgagccttgaattccacattcttcatcgctggcccatccacctccaagaggctgctgtcctccagctggccctctgacaccacatagttctgaataaaaaacatctttggcttccctgctagataagggcatgaatctcccatgaacatcctcctgatgtgatgcagggggagccctgagtgagtctgatccacaccatacacactctgggagcctcctcggctcaccaggacacacacaaagctgtcgtagtctcggtgctcgggcatacaggcaaattggccaagaatctgggatataccatgcatactgagatgcaagaatttctggacttcatagcccagggaagtgaaggtgtctcgaagaagctctgtctcattgccaatgcaatcgattatcaggcagattcctaggggcttgctcttcatcttgtatctctcttcaggtatgctcctgaagttatttgaaggatccttgagactcttttggattgctgcttggagaacattcctgtaacttgtccctgctccttgaacagactgcttgtacttctggatttttgtcttcaggtctattctgtggatgttctttaggcatttttctaataaatccagttgatctggggcaaccagatttagtttctccaactcaaccacaaggtccaagaaactcttctccttgcttatcttgcctcggcccatgtaatccttcatgaggaaaattaatgaggacacatcagatttatccaaatcctcaccaatctctgccatcagcactctatagtccgaaacaaggtgagggttcctgagcaggtgggtctccacagcttttctgtccatcttcaagatacgtttgagcaggtcaaatcgcctcactctgtagagcagttcagccaagtccccgacagacagcttacctctttcccgtaaaatatccagaaggtccctgacattaggtggaaccacatctatagcaacatcccggcacaaaaagagcagcatctccttctcatctgtatcaagtgcttcttcaacctgatggatgacttcagcagacatcctactcttagactagggaagctcacaagggtcttgcagtacagctccgggccagtcaacagaaagccagcaggcagtcaacttcatttctgagggctgacttcatttctttcagaatcctttccagtgggggagttcgtcctgtcgcggccggactctcctgccgctgccacctcagccttcgctcccctagacgccgggaaggcgcacccaagatggaggcaaagaaaccgaaagcctggaagcggacttggtgctgggcgatcgctgttcgcggcgcttctctcctacacctcctcccgtggtccttgttgtctcagctgtcactggacaaaagtccaatagccggcactcactgtgtgaggccgagtccccacccctagctccgggagtcccttttagttgagactcgtcggtgaggctgcaagctcgctgtttcctgctatggcttgtgt

SEQ ID NO: 15628 - RNA, 13363 nt, Homo sapiens
  source 1..13363: mol_type = other RNA
gctgggattacaggcatgagccactgtgcccagcctaaagcgtaataaactttcactgttgctctgaaacttgcctcggtccctccttctgccttatgcccctcagtcaaattctttcttctgaggaggaaagaattgaggttgctgcagatttaccaccagtaacttggataccgtccaccagtaacaacttccgttaagatggcaatacacctcaaatttatttttattttgagacagggtctcactctgttccccaggctggagtacagtggcacaatctcagctcactgaaacctccacctcccgggctcaagtgatcctcccacctcagccttccgagtagctggtactacaggcgcatgctaccatacccagctaatttttgtatttttagtagagacagggttttgccgtgttgcccaaggtggcctcaaattccttggctcaagcgatccaccatcctcagcctcccaaagtcctgggattacaggcatgagccactgcgcccagccaaacttatctttgtatgtttgttataggcaaaagtaccccaaggttaaggctcagcccaagaggtcaagtgggttcaggaaagaattcaagagcatgctgacagaataaagtgaaagcaagttcattaagaaagtaaaggaataaaagaatggctaccccataggaagagtagccctgatgggctgctgactggctatatttatggttgcttcttgactatacgctaaacaagaggtggcttattcatgagttttccaggaaagaagtggggaggtctggaccttttagaccatacagggtaacttctgaaagttgctatggcagttgtaaactatcatggtgctgtagaagtttcttttagcgtgctaatgtattataattaccatagaatgggcagcaaaggtaaccagaggtctcttctgtcaccatcatggttttggctggtttgggttggcctttctaccacatcctgtcttatcagcagggtcttacagggtcttgtggtcttgggaaaccagtcctgccaaactcctctcattcagtgtaatcactatcaaaattccagaggccctttttacataaatttgcaagtgaatcctaacagttatatgaaaatttagggaaaggtaaacccaatacagccctaacaattttgaaaaagaacaggccagttgcagtggctcacccctcagcactttgggaggtggaggtgggaggattgtttgaggccaggagtttgagaccagcctgggcaacatagcaaggcctcatctctacaaaagaaaaaagaagaacaacaacaacaacaaagttagaggactacatttctggattccaaaacttactacgaagttacaataatcaagacagtgtggtactaccataagatagagcaacagaattgagtccagaaataaacccttatagttagttgatttgtgataagtataaaataattctatagggaaaaaatagtattttcaataagtaatgctaagacaagtgaacatttatgtgcaaaagaatgaggctggatgcttatctcgcactgcatacacaaaaataactcaaaatgggtcaaagagctaaaatcataaaactttagaagaaaacataggggtaacacctcataggcaattgatttagacaatggttttttaggtatgacaccaaaagcataagcaataacataaaaaacagaaatcaagtgaacttcatcaaaatttaaaacttgtactgtatagtatccagaaagtgagaagacaatccatggaatgggagaatatattcacaaagattgtacctgataagaaactagtatccagaatattaaaaagaatgcttacaactcaacaataaaaagacaacccaccgggtgtggtggctcacgcctgtaatcctagcattttgggaggccgaggcaggcagatcacctgagttcaggagttcaagaccagcctggccaacatggcgaaaccctgtctctactaaaaatacaaaaattagccaggcgtgatggtgggtgcctgtaatcccagttactagggaggccgaggcaggagagtcgcttgaactcaggaggtggaggttgcagtgagccgagattgcaccactgcactccaacctgggcgacagagtgagattccatctcagaaaaataaaataaaataacgcagttttaaaatgagaaaggacttgaggccaggcacagtagctaatgtctgtaatgccagcactttgggaagccaaggcagtcagatcacctgaggccaggagttcgagaccagcctggccaacatggtgaaaccctgtctttactaaaaatacaaaaattggctgggcgcggtggctcacgcctgtaatcccagcactttgggaggccaaggcaggcggatcacgaggtcaggagatagagaccatcctggctaacacggtgaaaccctgtctctactaaaaatacaaaaaattagccgggcgtggtggagggcggctgtagtcccagatacttgggaggctgaggcaggagaatggcatgaacccaggaggcggagcttgcagtgagctgagattgcaccactgcactccagcctgggccacagagcgagactccgtctcaaaaaacaatacaaaaattagttgggcatggtggcgagctcctgtaaacccagctactcccaactactagggaggctgaggcaggagaatggcttgaacccagaaggcagaggttacagtgaatcaagataacgccactgcactccaccctgggcgacagagtgagactccgtctcaaaaacaaaaaaataaaaaaaacctcatacactgctggtgggaatataaaatgatgctactactttgaaaagcagtttggcagttcctcaaaaggctaaacatagagttactatatgatgagcactctcacttctaaggtatatgcccagaagaactgaaaacatatatccatataaaaattcatatacgaatattcatagcagcatcatccataatagcaaaaaagtggaaacagtctaaatttcgatcaactgatgaataaactaaatgcggtatatccacacaatagggtattattcagccataaaatgtaatgaagcactggtacactctatagcatagatgaaccttgaaacatgctaagtgaaggaagtcagacacgaaaggccacatgtttatttttataaaatatctagaacaggcaaatcatagagacagaaaatggattattgtttctagaggctgggggaagaggaggattagagtggcagctcactggtatggagtttctaggtagatggaaatgttctggaattagatagtggtgatgattgcacaactctgtaaatatactaaaatccactgcatcatttactttaaaggggcaaattttatggcttgtgaattacatttcaataaaaagaagatgaggaaacctaggatatgtcacaatcccatgccacaaactacttacacttccaatataaaaactatatcaacaatagtttacatcacgttcattgcttgctaaagtaaggtcatgaatgtatcaaaatattttataaaagttaaaatttaggagatccatcatttctcttttcaatccatcactgattcattcaatatatatttatgtgtatgccaggctcttcatcaggtaaagtgtttaggagagatataaagataaaactgatgagaattctgcacttgagctacagcatactttccaagaattacagcatgagatataaaatgaaaagaaggcttggaggagattcacacgaaatagtactgttcaggagagggggcgataattccaatggaagagataactgacttcatggaggatagaaggagatggtatttgaactgcccttgaagtatggttatattttggggatgtggagatgtggggtagggtgatatgctggggttccagatggtccagaaatatacaatcaccagaaccaaagatccagaggtaggagatatgagctgttcaatttggctgagctaacagtgtttggagtgggatcttgaagaagctgaaaatgaagataccaactagacagtcagagaaagacttccaatgtttgactgaactgcaattttattgtgtatgcattgaagaatctttttttttttttttgtattctctaaagatttttaaaatattttaagttctggatacaagtgcaggatgtgcgggtttgttacataggtaaacgtgtcccatggtggtttgctgcacctatcaacctatcacctaggtattaagccccacatgcattagctagttatcctgatgctctccccgctacggcccctgcatcaggccccagtgtgtgttgatctcatccctgtgtccgtgtgttctcattgttcagcttccgcttacaagtgagaacatgtggtgtttggtttcctgctcctctgttagtttgctgaggataatggcttccagcttcatccatgtccctgcaaaggacatgatctcattccttttttaaaaaaaaaaacaaaattatttccataggtgtttggggaacaggtggtatctggttacatgcgtaagtaattaagtggttacttgtgagattctggtgcacccatcacctgagcagtatacactgaacccaatttgtattcttttatccttcacccccctcccaccctttcccctaagtccccaaagtccattgtatccttcttatgcctttgcatcctcatagcttatctcccacttatgagtgagaacatacaatgtttggttttccattcctcagttacttcctttagagtaatagtctccaggttgctgtgaatgtcattaattcattcctttttatggctgagtagtgtttaggtgaggttatttgtaagtaattaatattgagtaaataagattcatccatagtggcaaagccacataacttctaagtatcttaaactatatctaaatggtaccaaaacatgcagtcaattctaaaagctcagctaatgatatttcataatataggaaaatattcacaacatatttttgtgtaaaaaaaagcagacttcaaaatggaatatgcattatgattccaatcatgtaaaagctatacatgaacacatacaaagattaacagatataaacaaatggaagaatgaatggagagatagatgatagacagattgagtggtggtggagaataacagatttaaaaagaaattgtgcctttctatattttcaaaaccatttaaataagtattacctttggagttagaaaatgatatgtattttaaatccataattcaactacttatctatatgatgtcaaactggattaggctgaattatcagcaagtgaataaaacagttccttcatccatggagaaacatccatttatgacattcttggaattcctcttgttagaattctttatgaatttaaaatagaaacatggccagactcaagatttcaatacaaacattactttttcacgttcagtaataaccaattaaaagaattaatgaaaaatctgattcactgtatcaccaaaagctgtaatggctgcactgcacagtattccatggtgtatatgtaccacattttctttatccagtctatctttgatgggcatttgctattgtgtctttgctattgtgaagagtgctgcaatgaacaaaaatgtgcatgtatctttataataaaatggtttatattcctttgggtatatacccagtaatgggattgctgggacaaatagtatttctagttctagatctttgaggaatagccacacacacttccacaacggttgaactaatttacattcccaccaacaatgtaaaagtgttcctacttctccacagcctcgccagcatctgttgttttttgactttttaataatcaccattctgaccggcatgagatggtatctcattgtggttctcctttgcatttctctaatgatcagtaaggttgagcttttttttatatgtttgttggccacataaatgtcttcttttgagaagtgtctgttcatgtcctttgtccactttttgatggggttgtttttttccttgtaaatttgttttaagttccttgtaggttctggatattagacctttgtcagatggatagattgcaaaaatgttctcccattctgtaggttgcctgttcactctaatgatagtttcttttgctgtgcaggagctctttagtttaattagatcccatttgtaatttttgcttttgttgcaattgcttttgatgtttttgtcatgaaacctttgcttgtgcctatgtcttgaatggtattaaatagattttcttctagggtttttatagttttaggttttacattaagtctttaatcttgagttaatttttgtataaggtgtaaggaaggggtcagtttcaattttctgcatatggctagccagttttcccagcaccatttattaaatagggaatcttttccccattgcttgtttttgtcaggtttgtcgatgatcagatggctgtagatgtgtggtcttctttctctggtctctattctgttccattggtctatgtgtctgtttttgtaccagtaccatgccattttggctactgtagccttgcagtatactttgaagttgggtagtgtgatgcttccagctttgttctttttgcttattgttgtcttggttatacgggctcttttttggttccatttgaattttaaagtagtttttttctaattctgtgaagaatgtcaatagtagtttaatgggaatagcaatgaacctataaattactttgggtagtatggccattttcatgatattgattcttcctatccacgagaatggaatgttttttcatttgtgtcctctcttatttccttgagcagtggtttgtagttctccttgaagagatccttcacatcttattagctgtattcctaggtattttattctctttctagcaactgtgaatgggagttcattcatgatttggctctctgcttgtgtattgttggtgtatagaatgcttgtgatttctgcacattgattttgtatcctgagactttgctgaagttgcttatcagcttaaggaacttttgggtggagataatggggttttctagatatagtatcatgtcatctgcaaacacagttttacttcctcttttcctatttgaataccccttatttgtttctcttgcctgattttcttggccagaacttccaatactatgttaaataggagtggtgagacggcatccctgtcttgtgccagttttcaaggggaatgcttccagcttttgcccattcagtatgataatggctgtgggtttgtcataaatggttattattttgagatattttccatcaatacctagtttattgagagtttttaacatgaagcaacgttgaattttattgaaggccttttctgtatctattgagataatcatgtggtttttgtctttagttctgtttatgtgatgaattatgtttcttgatttgcgtatgttgaaccagccttgcatcccagggatgaagccaacattccaaacattttatttattatttatttatttatttatttttgagacagagtctcgcactgtcgcccaggctggagtgcagtggcaagatctcagctcgctgcaagctccacctcccaggttcatgccgttctcttgcctcggcctcccaaatagcagggactacaggcgaccgccacaacgcctggctaattttttgtatttttagtagagacggggttttacatgttagccaggatggtcttgatctcctgacctcgtgatccgcccgccttggcctcccaaagggctgggattataggcgtgagccaccgcacccggcctccaaacattttaatctcataacaatgcatcacttgggttaactaggttgagataaatataaactgtcaattttttttcccctcacataaaagtccagaggtaggtaattagggctgacacagtgattccagtgattctgctccttcgtgccctcatccaacaaggcttcttgctgctcactacccagctacccctacgtgtggcccgtatcttcatggttcaagatggcagctagagctgctaggtagttaagatctctctcacacactttccttctgtcataattaacacagggttttagctcatgaggccaagcatacacattacttcccactggcacccctatgtaatattaaatgcaaagataccctcaggagtcctgtgctcaaaacaagtacaaaataactttttgttgttgtttgtggtgctggtggttttatttatttattttttctgaaacagggtctcactctgtctcccatgctgaagtgcagtggtgtgatcacagctcatcacaaccttgacctctctgggctcaggggatccactcacttcagcctcccaagtagctgggactacaggaacacgccaccacgctcagctaaattttgtctttttttgtagagatggagtcttgctatgttgcccaggctggtctcaaactcctgggctcaagtgatcagtccacctcagcctcccaaagtactcagattataggtatgagccaccatggcatcaaaataacttggaaagtaggaataattgcttgttgttcctgaaaactgtctcttcgacacttttcagactctgttacatgatcatgacaaaatatacacaaatagacatacagatacacatcagttaaaacctcaagaaatagaaaaataaataaatcataaaatatttaaaaagtggtattctgacacactgcccagaggtacccctgttcagcaattttaaaaaattttaaaaatagccctctccccctccctctcttctccctctccccacggtctccctctgatgccgagccgaagctggactgtactgctgccatctcggctcactgcagcctccctgcctgattctcccgcctcggcctgccgcgtgcctgccattgcgggcgccgccacgcctgactggttttcgtatttttttggtggagacagggtttcactgtgttggccgggctggtctccagctcctgactgcgagtgatctgccagcctcggcctcccgaggtgccgggattgcgggcagagtctcgtccactcagtgctcaatgttgcccaggctggagtgcagtggtgtgatctcagctggctacggcctccgcctcccagccgcctgccttggccccccagggtgccgagattacagcttctgcccggccgccaccccgtctgggatgaagtgaggagcgtctctgcccggccgcccatcgtctgagatgtggggagcgcctctgccccgcccccccgtctgggatgtgaggagcttctctgcccggccaccccgtctgagaagtgaggagcccctccgcccgcagctgccccgtctgagaagtgaggagcccctccgcccgacagccaccctgtctgggaagtgaggagcgtctccgcccagcagccaccccgtctgagaagtgaggagcccctccgcctggcagccgccccgtccgggagggaggcgtgggggtcagcccccgcccggccagccgccccgtcggggagggaggtggggggtcagcccccgcccggccagctatcccgtccgggagggaggtggggggcgcgtccgcctggccgccccatctgggaagtgaggagcccctctgcccagccgccaccccgtctgggaggtgtacccaacagctcattgagaacaggccatgatgacgatggcggttttgtggaatagaaaagggggaaaggtggggaaaagatagagaaatcagattgttgctgtgtctgtgtagaaagaagtagacatgggagacttcattttgttctgtactaagaaaaattcttctgccttaggatgctgttgatctatgaccttacccccaaccctgtgctctctgaaacatgtgctgtgtccactcagggttaaatggattaagggcagtgcaagatgtgctttgttaaacagatgcttgaaggcagcatgctccttaagagtcatcaccactccctaatctcaagtacccagggacacaaacactgcggaaggccgcagggtcctctgcctaggaaaaccagagacctttgttcacttgtttatctgctgaccttccctccactattgtcctgtgaccctgccaaatcaccctctgtgagaaacacccaagaatgatcaattaaaaaaaaaaaatttaaaaataataataggccaggtgcagtggctcacacctgtaatcccagcactttgggaggccgaggctggtgaatcacctgaggtcaggagttcaagaccacgctggccaacatggtggaaaccctgtctccactaaaaatacaaaaattagccgggtgtggtggcaggagcctgtaatcccagctactcgggaggctgaggcaggagaatcgcttgaacccagaaggcagaggttgcaatgagccaagatgatgccactgcactccagcctgggcagcagaatgaaactctgtctcaataataataataataataataataataataataataataataataagcaactctaatgatatttcaaacaatggtccccttttaggtcacactatcaaatcagagaaagatatacttgactagctgtaaaatgcaatttgaggtctaggtgaatgaacaagtaacctctaaatcataaggctattgttacaaactgaatgtttgtattccccccagaattcaaaggggagacagtatccccaaagtgacagtatcagaaggtggggcctttgggaggtaattaggtgatgagggtagagccctcatgaatggaatttgtgcccttaaagatatacttgagagtttgcatcctctttttctgccatgtgagaacatcaaaagactgacatctggtaagatctggaagcatgccttaccagacaccagatatgctaccacttagatgttggatttcccagcctccggaactgtgagaaataactgctgtttaagtcacctggtctatggtaatttggtatagttgcccaaatggactgtgatggttaatactgagtatcaacttgattgaatagaaggatgcaaagtgttcccgggtacatctgtgagggtgctgccaaaggagatttaacatttgagtcagtggactgggaaaggcagaccatcctcaatctgggtgggcaccatctaatcagctgccagcactgccagaataaaagcaggcaaaacatggaaagactagactggtgtagtcttctggcctccatctttctctcatgctgaatgcttcctgccctcaaacattggactccaagttcttcagctttgggacttgaattggcttccttgcttgcagatgacctattgtgggacctaaccctgtgatcatgtgagtcaatactccttaataaactcccctttttatatacatgtatcctattagttctgtccctctagagaaacatgactaatacattgagtaagatagttcctgtcctttttttttttttttaaagagatgggatcttgctatattgcccaggttggtatgcagtggctattcgtaggcacaatcacagcatgctatgaccctgaactcctgggttcaaaagatcctcccacctcagcctcccaagtaactgggaatacaggtacccacacccacacccagctaatttttgtatttttactagggacagcgtttaccatgttggccaggctggtctcgaactcctgacctgaagtgatctgccctccttggcctcccaaagtgctgggattacaggtgtgagccactacgcccagccttttggtttcttatgtgtaggagaggataagtttctttctcagagtgtgctgcagccagacataatatttctccttggcagaaactctgctgttccaatcatacatgtagccattgagttcaatgtgaagatccaggagtgggcgttttctttcttgtctcagtttctgggagaggcactgcaggtacagggatggtgagctgtgagactgctccagcagggacatgtccgcagtacacaggctccagaagaagtcagcttctcggtgaactgtgcacagccctcgcttctgagccttgaattccacattcttcatcgctggcccatccacctccaagaggctgctgtcctccagctggccctctgacaccacatagttctgaataaaaaacatctttggcttccctgctagataagggcatgaatctcccatgaacatcctcctgatgtgatgcagggggagccctgagtgagtctgatccacaccatacacactctgggagcctcctcggctcaccaggacacacacaaagctgtcgtagtctcggtgctcgggcatacaggcaaattggccaagaatctgggatataccatgcatactgagatgcaagaatttctggacttcatagcccagggaagtgaaggtgtctcgaagaagctctgtctcattgccaatgcaatcgattatcaggcagattcctaggggcttgctcttcatcttgtatctctcttcaggtatgctctgaggcaaaaaagcttctgattcctgaatggatttcttcactggttcttgttgagcgccaagctgttccttaagtctttgttctttacttctcccattatggagcctgaagttatttgaaggatccttgagactcttttggattgctgcttggagaacattcctgtaacttgtccctgctccttgaacagactgcttgtacttctggatttttgtcttcaggtctattctgtggatgttctttaggcatttttctaataaatccagttgatctggggcaaccagatttagtttctccaactcaaccacaaggtccaagaaactcttctccttgcttatcttgcctcggcccatgtaatccttcatgaggaaaattaatgaggacacatcagatttatccaaatcctcaccaatctctgccatcagcactcgtcctgtcgcggccggactctcctgccgctgccacctcagccttcgctcccctagacgccgggaaggcgcacccaagatggaggcaaagaaaccgaaagcctggaagcggacttggtgctgggcgatcgctgttcgcggcgcttctctcctacacctcctcccgtggtccttgttgtctcagctgtcactggacaaaagtccaatagccggcactcactgtgtgaggccgagtccccacccctagctccgggagtcccttttagttgagactcgtcggtgaggctgcaagctcgctgtttcctgctatggcttgtgt

SEQ ID NO: 15629 - RNA, 13781 nt, Homo sapiens
  source 1..13781: mol_type = other RNA
gctgggattacaggcatgagccactgtgcccagcctaaagcgtaataaactttcactgttgctctgaaacttgcctcggtccctccttctgccttatgcccctcagtcaaattctttcttctgaggaggaaagaattgaggttgctgcagatttaccaccagtaacttggataccgtccaccagtaacaacttccgttaagatggcaatacacctcaaatttatttttattttgagacagggtctcactctgttccccaggctggagtacagtggcacaatctcagctcactgaaacctccacctcccgggctcaagtgatcctcccacctcagccttccgagtagctggtactacaggcgcatgctaccatacccagctaatttttgtatttttagtagagacagggttttgccgtgttgcccaaggtggcctcaaattccttggctcaagcgatccaccatcctcagcctcccaaagtcctgggattacaggcatgagccactgcgcccagccaaacttatctttgtatgtttgttataggcaaaagtaccccaaggttaaggctcagcccaagaggtcaagtgggttcaggaaagaattcaagagcatgctgacagaataaagtgaaagcaagttcattaagaaagtaaaggaataaaagaatggctaccccataggaagagtagccctgatgggctgctgactggctatatttatggttgcttcttgactatacgctaaacaagaggtggcttattcatgagttttccaggaaagaagtggggaggtctggaccttttagaccatacagggtaacttctgaaagttgctatggcagttgtaaactatcatggtgctgtagaagtttcttttagcgtgctaatgtattataattaccatagaatgggcagcaaaggtaaccagaggtctcttctgtcaccatcatggttttggctggtttgggttggcctttctaccacatcctgtcttatcagcagggtcttacagggtcttgtggtcttgggaaaccagtcctgccaaactcctctcattcagtgtaatcactatcaaaattccagaggccctttttacataaatttgcaagtgaatcctaacagttatatgaaaatttagggaaaggtaaacccaatacagccctaacaattttgaaaaagaacaggccagttgcagtggctcacccctcagcactttgggaggtggaggtgggaggattgtttgaggccaggagtttgagaccagcctgggcaacatagcaaggcctcatctctacaaaagaaaaaagaagaacaacaacaacaacaaagttagaggactacatttctggattccaaaacttactacgaagttacaataatcaagacagtgtggtactaccataagatagagcaacagaattgagtccagaaataaacccttatagttagttgatttgtgataagtataaaataattctatagggaaaaaatagtattttcaataagtaatgctaagacaagtgaacatttatgtgcaaaagaatgaggctggatgcttatctcgcactgcatacacaaaaataactcaaaatgggtcaaagagctaaaatcataaaactttagaagaaaacataggggtaacacctcataggcaattgatttagacaatggttttttaggtatgacaccaaaagcataagcaataacataaaaaacagaaatcaagtgaacttcatcaaaatttaaaacttgtactgtatagtatccagaaagtgagaagacaatccatggaatgggagaatatattcacaaagattgtacctgataagaaactagtatccagaatattaaaaagaatgcttacaactcaacaataaaaagacaacccaccgggtgtggtggctcacgcctgtaatcctagcattttgggaggccgaggcaggcagatcacctgagttcaggagttcaagaccagcctggccaacatggcgaaaccctgtctctactaaaaatacaaaaattagccaggcgtgatggtgggtgcctgtaatcccagttactagggaggccgaggcaggagagtcgcttgaactcaggaggtggaggttgcagtgagccgagattgcaccactgcactccaacctgggcgacagagtgagattccatctcagaaaaataaaataaaataacgcagttttaaaatgagaaaggacttgaggccaggcacagtagctaatgtctgtaatgccagcactttgggaagccaaggcagtcagatcacctgaggccaggagttcgagaccagcctggccaacatggtgaaaccctgtctttactaaaaatacaaaaattggctgggcgcggtggctcacgcctgtaatcccagcactttgggaggccaaggcaggcggatcacgaggtcaggagatagagaccatcctggctaacacggtgaaaccctgtctctactaaaaatacaaaaaattagccgggcgtggtggagggcggctgtagtcccagatacttgggaggctgaggcaggagaatggcatgaacccaggaggcggagcttgcagtgagctgagattgcaccactgcactccagcctgggccacagagcgagactccgtctcaaaaaacaatacaaaaattagttgggcatggtggcgagctcctgtaaacccagctactcccaactactagggaggctgaggcaggagaatggcttgaacccagaaggcagaggttacagtgaatcaagataacgccactgcactccaccctgggcgacagagtgagactccgtctcaaaaacaaaaaaataaaaaaaacctcatacactgctggtgggaatataaaatgatgctactactttgaaaagcagtttggcagttcctcaaaaggctaaacatagagttactatatgatgagcactctcacttctaaggtatatgcccagaagaactgaaaacatatatccatataaaaattcatatacgaatattcatagcagcatcatccataatagcaaaaaagtggaaacagtctaaatttcgatcaactgatgaataaactaaatgcggtatatccacacaatagggtattattcagccataaaatgtaatgaagcactggtacactctatagcatagatgaaccttgaaacatgctaagtgaaggaagtcagacacgaaaggccacatgtttatttttataaaatatctagaacaggcaaatcatagagacagaaaatggattattgtttctagaggctgggggaagaggaggattagagtggcagctcactggtatggagtttctaggtagatggaaatgttctggaattagatagtggtgatgattgcacaactctgtaaatatactaaaatccactgcatcatttactttaaaggggcaaattttatggcttgtgaattacatttcaataaaaagaagatgaggaaacctaggatatgtcacaatcccatgccacaaactacttacacttccaatataaaaactatatcaacaatagtttacatcacgttcattgcttgctaaagtaaggtcatgaatgtatcaaaatattttataaaagttaaaatttaggagatccatcatttctcttttcaatccatcactgattcattcaatatatatttatgtgtatgccaggctcttcatcaggtaaagtgtttaggagagatataaagataaaactgatgagaattctgcacttgagctacagcatactttccaagaattacagcatgagatataaaatgaaaagaaggcttggaggagattcacacgaaatagtactgttcaggagagggggcgataattccaatggaagagataactgacttcatggaggatagaaggagatggtatttgaactgcccttgaagtatggttatattttggggatgtggagatgtggggtagggtgatatgctggggttccagatggtccagaaatatacaatcaccagaaccaaagatccagaggtaggagatatgagctgttcaatttggctgagctaacagtgtttggagtgggatcttgaagaagctgaaaatgaagataccaactagacagtcagagaaagacttccaatgtttgactgaactgcaattttattgtgtatgcattgaagaatctttttttttttttttgtattctctaaagatttttaaaatattttaagttctggatacaagtgcaggatgtgcgggtttgttacataggtaaacgtgtcccatggtggtttgctgcacctatcaacctatcacctaggtattaagccccacatgcattagctagttatcctgatgctctccccgctacggcccctgcatcaggccccagtgtgtgttgatctcatccctgtgtccgtgtgttctcattgttcagcttccgcttacaagtgagaacatgtggtgtttggtttcctgctcctctgttagtttgctgaggataatggcttccagcttcatccatgtccctgcaaaggacatgatctcattccttttttaaaaaaaaaaacaaaattatttccataggtgtttggggaacaggtggtatctggttacatgcgtaagtaattaagtggttacttgtgagattctggtgcacccatcacctgagcagtatacactgaacccaatttgtattcttttatccttcacccccctcccaccctttcccctaagtccccaaagtccattgtatccttcttatgcctttgcatcctcatagcttatctcccacttatgagtgagaacatacaatgtttggttttccattcctcagttacttcctttagagtaatagtctccaggttgctgtgaatgtcattaattcattcctttttatggctgagtagtgtttaggtgaggttatttgtaagtaattaatattgagtaaataagattcatccatagtggcaaagccacataacttctaagtatcttaaactatatctaaatggtaccaaaacatgcagtcaattctaaaagctcagctaatgatatttcataatataggaaaatattcacaacatatttttgtgtaaaaaaaagcagacttcaaaatggaatatgcattatgattccaatcatgtaaaagctatacatgaacacatacaaagattaacagatataaacaaatggaagaatgaatggagagatagatgatagacagattgagtggtggtggagaataacagatttaaaaagaaattgtgcctttctatattttcaaaaccatttaaataagtattacctttggagttagaaaatgatatgtattttaaatccataattcaactacttatctatatgatgtcaaactggattaggctgaattatcagcaagtgaataaaacagttccttcatccatggagaaacatccatttatgacattcttggaattcctcttgttagaattctttatgaatttaaaatagaaacatggccagactcaagatttcaatacaaacattactttttcacgttcagtaataaccaattaaaagaattaatgaaaaatctgattcactgtatcaccaaaagctgtaatggctgcactgcacagtattccatggtgtatatgtaccacattttctttatccagtctatctttgatgggcatttgctattgtgtctttgctattgtgaagagtgctgcaatgaacaaaaatgtgcatgtatctttataataaaatggtttatattcctttgggtatatacccagtaatgggattgctgggacaaatagtatttctagttctagatctttgaggaatagccacacacacttccacaacggttgaactaatttacattcccaccaacaatgtaaaagtgttcctacttctccacagcctcgccagcatctgttgttttttgactttttaataatcaccattctgaccggcatgagatggtatctcattgtggttctcctttgcatttctctaatgatcagtaaggttgagcttttttttatatgtttgttggccacataaatgtcttcttttgagaagtgtctgttcatgtcctttgtccactttttgatggggttgtttttttccttgtaaatttgttttaagttccttgtaggttctggatattagacctttgtcagatggatagattgcaaaaatgttctcccattctgtaggttgcctgttcactctaatgatagtttcttttgctgtgcaggagctctttagtttaattagatcccatttgtaatttttgcttttgttgcaattgcttttgatgtttttgtcatgaaacctttgcttgtgcctatgtcttgaatggtattaaatagattttcttctagggtttttatagttttaggttttacattaagtctttaatcttgagttaatttttgtataaggtgtaaggaaggggtcagtttcaattttctgcatatggctagccagttttcccagcaccatttattaaatagggaatcttttccccattgcttgtttttgtcaggtttgtcgatgatcagatggctgtagatgtgtggtcttctttctctggtctctattctgttccattggtctatgtgtctgtttttgtaccagtaccatgccattttggctactgtagccttgcagtatactttgaagttgggtagtgtgatgcttccagctttgttctttttgcttattgttgtcttggttatacgggctcttttttggttccatttgaattttaaagtagtttttttctaattctgtgaagaatgtcaatagtagtttaatgggaatagcaatgaacctataaattactttgggtagtatggccattttcatgatattgattcttcctatccacgagaatggaatgttttttcatttgtgtcctctcttatttccttgagcagtggtttgtagttctccttgaagagatccttcacatcttattagctgtattcctaggtattttattctctttctagcaactgtgaatgggagttcattcatgatttggctctctgcttgtgtattgttggtgtatagaatgcttgtgatttctgcacattgattttgtatcctgagactttgctgaagttgcttatcagcttaaggaacttttgggtggagataatggggttttctagatatagtatcatgtcatctgcaaacacagttttacttcctcttttcctatttgaataccccttatttgtttctcttgcctgattttcttggccagaacttccaatactatgttaaataggagtggtgagacggcatccctgtcttgtgccagttttcaaggggaatgcttccagcttttgcccattcagtatgataatggctgtgggtttgtcataaatggttattattttgagatattttccatcaatacctagtttattgagagtttttaacatgaagcaacgttgaattttattgaaggccttttctgtatctattgagataatcatgtggtttttgtctttagttctgtttatgtgatgaattatgtttcttgatttgcgtatgttgaaccagccttgcatcccagggatgaagccaacattccaaacattttatttattatttatttatttatttatttttgagacagagtctcgcactgtcgcccaggctggagtgcagtggcaagatctcagctcgctgcaagctccacctcccaggttcatgccgttctcttgcctcggcctcccaaatagcagggactacaggcgaccgccacaacgcctggctaattttttgtatttttagtagagacggggttttacatgttagccaggatggtcttgatctcctgacctcgtgatccgcccgccttggcctcccaaagggctgggattataggcgtgagccaccgcacccggcctccaaacattttaatctcataacaatgcatcacttgggttaactaggttgagataaatataaactgtcaattttttttcccctcacataaaagtccagaggtaggtaattagggctgacacagtgattccagtgattctgctccttcgtgccctcatccaacaaggcttcttgctgctcactacccagctacccctacgtgtggcccgtatcttcatggttcaagatggcagctagagctgctaggtagttaagatctctctcacacactttccttctgtcataattaacacagggttttagctcatgaggccaagcatacacattacttcccactggcacccctatgtaatattaaatgcaaagataccctcaggagtcctgtgctcaaaacaagtacaaaataactttttgttgttgtttgtggtgctggtggttttatttatttattttttctgaaacagggtctcactctgtctcccatgctgaagtgcagtggtgtgatcacagctcatcacaaccttgacctctctgggctcaggggatccactcacttcagcctcccaagtagctgggactacaggaacacgccaccacgctcagctaaattttgtctttttttgtagagatggagtcttgctatgttgcccaggctggtctcaaactcctgggctcaagtgatcagtccacctcagcctcccaaagtactcagattataggtatgagccaccatggcatcaaaataacttggaaagtaggaataattgcttgttgttcctgaaaactgtctcttcgacacttttcagactctgttacatgatcatgacaaaatatacacaaatagacatacagatacacatcagttaaaacctcaagaaatagaaaaataaataaatcataaaatatttaaaaagtggtattctgacacactgcccagaggtacccctgttcagcaattttaaaaaattttaaaaatagccctctccccctccctctcttctccctctccccacggtctccctctgatgccgagccgaagctggactgtactgctgccatctcggctcactgcagcctccctgcctgattctcccgcctcggcctgccgcgtgcctgccattgcgggcgccgccacgcctgactggttttcgtatttttttggtggagacagggtttcactgtgttggccgggctggtctccagctcctgactgcgagtgatctgccagcctcggcctcccgaggtgccgggattgcgggcagagtctcgtccactcagtgctcaatgttgcccaggctggagtgcagtggtgtgatctcagctggctacggcctccgcctcccagccgcctgccttggccccccagggtgccgagattacagcttctgcccggccgccaccccgtctgggatgaagtgaggagcgtctctgcccggccgcccatcgtctgagatgtggggagcgcctctgccccgcccccccgtctgggatgtgaggagcttctctgcccggccaccccgtctgagaagtgaggagcccctccgcccgcagctgccccgtctgagaagtgaggagcccctccgcccgacagccaccctgtctgggaagtgaggagcgtctccgcccagcagccaccccgtctgagaagtgaggagcccctccgcctggcagccgccccgtccgggagggaggcgtgggggtcagcccccgcccggccagccgccccgtcggggagggaggtggggggtcagcccccgcccggccagctatcccgtccgggagggaggtggggggcgcgtccgcctggccgccccatctgggaagtgaggagcccctctgcccagccgccaccccgtctgggaggtgtacccaacagctcattgagaacaggccatgatgacgatggcggttttgtggaatagaaaagggggaaaggtggggaaaagatagagaaatcagattgttgctgtgtctgtgtagaaagaagtagacatgggagacttcattttgttctgtactaagaaaaattcttctgccttaggatgctgttgatctatgaccttacccccaaccctgtgctctctgaaacatgtgctgtgtccactcagggttaaatggattaagggcagtgcaagatgtgctttgttaaacagatgcttgaaggcagcatgctccttaagagtcatcaccactccctaatctcaagtacccagggacacaaacactgcggaaggccgcagggtcctctgcctaggaaaaccagagacctttgttcacttgtttatctgctgaccttccctccactattgtcctgtgaccctgccaaatcaccctctgtgagaaacacccaagaatgatcaattaaaaaaaaaaaatttaaaaataataataggccaggtgcagtggctcacacctgtaatcccagcactttgggaggccgaggctggtgaatcacctgaggtcaggagttcaagaccacgctggccaacatggtggaaaccctgtctccactaaaaatacaaaaattagccgggtgtggtggcaggagcctgtaatcccagctactcgggaggctgaggcaggagaatcgcttgaacccagaaggcagaggttgcaatgagccaagatgatgccactgcactccagcctgggcagcagaatgaaactctgtctcaataataataataataataataataataataataataataataataagcaactctaatgatatttcaaacaatggtccccttttaggtcacactatcaaatcagagaaagatatacttgactagctgtaaaatgcaatttgaggtctaggtgaatgaacaagtaacctctaaatcataaggctattgttacaaactgaatgtttgtattccccccagaattcaaaggggagacagtatccccaaagtgacagtatcagaaggtggggcctttgggaggtaattaggtgatgagggtagagccctcatgaatggaatttgtgcccttaaagatatacttgagagtttgcatcctctttttctgccatgtgagaacatcaaaagactgacatctggtaagatctggaagcatgccttaccagacaccagatatgctaccacttagatgttggatttcccagcctccggaactgtgagaaataactgctgtttaagtcacctggtctatggtaatttggtatagttgcccaaatggactgtgatggttaatactgagtatcaacttgattgaatagaaggatgcaaagtgttcccgggtacatctgtgagggtgctgccaaaggagatttaacatttgagtcagtggactgggaaaggcagaccatcctcaatctgggtgggcaccatctaatcagctgccagcactgccagaataaaagcaggcaaaacatggaaagactagactggtgtagtcttctggcctccatctttctctcatgctgaatgcttcctgccctcaaacattggactccaagttcttcagctttgggacttgaattggcttccttgcttgcagatgacctattgtgggacctaaccctgtgatcatgtgagtcaatactccttaataaactcccctttttatatacatgtatcctattagttctgtccctctagagaaacatgactaatacattgagtaagatagttcctgtcctttttttttttttttaaagagatgggatcttgctatattgcccaggttggtatgcagtggctattcgtaggcacaatcacagcatgctatgaccctgaactcctgggttcaaaagatcctcccacctcagcctcccaagtaactgggaatacaggtacccacacccacacccagctaatttttgtatttttactagggacagcgtttaccatgttggccaggctggtctcgaactcctgacctgaagtgatctgccctccttggcctcccaaagtgctgggattacaggtgtgagccactacgcccagccttttggtttcttatgtgtaggagaggataagtttctttctcagagtgtgctgcagccagacataatatttctccttggcagaaactctgctgttccaatcatacatgtagccattgagttcaatgtgaagatccaggagtgggcgttttctttcttgtctcagtttctgggagaggcactgcaggtacagggatggtgagctgtgagactgctccagcagggacatgtccgcagtacacaggctccagaagaagtcagcttctcggtgaactgtgcacagccctcgcttctgagccttgaattccacattcttcatcgctggcccatccacctccaagaggctgctgtcctccagctggccctctgacaccacatagttctgaataaaaaacatctttggcttccctgctagataagggcatgaatctcccatgaacatcctcctgatgtgatgcagggggagccctgagtgagtctgatccacaccatacacactctgggagcctcctcggctcaccaggacacacacaaagctgtcgtagtctcggtgctcgggcatacaggcaaattggccaagaatctgggatataccatgcatactgagatgcaagaatttctggacttcatagcccagggaagtgaaggtgtctcgaagaagctctgtctcattgccaatgcaatcgattatcaggcagattcctaggggcttgctcttcatcttgtatctctcttcaggtatgctctgaggcaaaaaagcttctgattcctgaatggatttcttcactggttcttgttgagcgccaagctgttccttaagtctttgttctttacttctcccattatggagcctgaagttatttgaaggatccttgagactcttttggattgctgcttggagaacattcctgtaacttgtccctgctccttgaacagactgcttgtacttctggatttttgtcttcaggtctattctgtggatgttctttaggcatttttctaataaatccagttgatctggggcaaccagatttagtttctccaactcaaccacaaggtccaagaaactcttctccttgcttatcttgcctcggcccatgtaatccttcatgaggaaaattaatgaggacacatcagatttatccaaatcctcaccaatctctgccatcagcactctatagtccgaaacaaggtgagggttcctgagcaggtgggtctccacagcttttctgtccatcttcaagatacgtttgagcaggtcaaatcgcctcactctgtagagcagttcagccaagtccccgacagacagcttacctctttcccgtaaaatatccagaaggtccctgacattaggtggaaccacatctatagcaacatcccggcacaaaaagagcagcatctccttctcatctgtatcaagtgcttcttcaacctgatggatgacttcagcagacatcctactcttagactagggaagctcacaagggtcttgcagtacagctccgggccagtcaacagaaagccagcaggcagtcaacttcatttctgagggctgacttcatttctttcagaatcctttccagtgggggagttcgtcctgtcgcggccggactctcctgccgctgccacctcagccttcgctcccctagacgccgggaaggcgcacccaagatggaggcaaagaaaccgaaagcctggaagcggacttggtgctgggcgatcgctgttcgcggcgcttctctcctacacctcctcccgtggtccttgttgtctcagctgtcactggacaaaagtccaatagccggcactcactgtgtgaggccgagtccccacccctagctccgggagtcccttttagttgagactcgtcggtgaggctgcaagctcgctgtttcctgctatggcttgtgt

SEQ ID NO: 15630 - RNA, 13649 nt, Homo sapiens
  source 1..13649: mol_type = other RNA
gctgggattacaggcatgagccactgtgcccagcctaaagcgtaataaactttcactgttgctctgaaacttgcctcggtccctccttctgccttatgcccctcagtcaaattctttcttctgaggaggaaagaattgaggttgctgcagatttaccaccagtaacttggataccgtccaccagtaacaacttccgttaagatggcaatacacctcaaatttatttttattttgagacagggtctcactctgttccccaggctggagtacagtggcacaatctcagctcactgaaacctccacctcccgggctcaagtgatcctcccacctcagccttccgagtagctggtactacaggcgcatgctaccatacccagctaatttttgtatttttagtagagacagggttttgccgtgttgcccaaggtggcctcaaattccttggctcaagcgatccaccatcctcagcctcccaaagtcctgggattacaggcatgagccactgcgcccagccaaacttatctttgtatgtttgttataggcaaaagtaccccaaggttaaggctcagcccaagaggtcaagtgggttcaggaaagaattcaagagcatgctgacagaataaagtgaaagcaagttcattaagaaagtaaaggaataaaagaatggctaccccataggaagagtagccctgatgggctgctgactggctatatttatggttgcttcttgactatacgctaaacaagaggtggcttattcatgagttttccaggaaagaagtggggaggtctggaccttttagaccatacagggtaacttctgaaagttgctatggcagttgtaaactatcatggtgctgtagaagtttcttttagcgtgctaatgtattataattaccatagaatgggcagcaaaggtaaccagaggtctcttctgtcaccatcatggttttggctggtttgggttggcctttctaccacatcctgtcttatcagcagggtcttacagggtcttgtggtcttgggaaaccagtcctgccaaactcctctcattcagtgtaatcactatcaaaattccagaggccctttttacataaatttgcaagtgaatcctaacagttatatgaaaatttagggaaaggtaaacccaatacagccctaacaattttgaaaaagaacaggccagttgcagtggctcacccctcagcactttgggaggtggaggtgggaggattgtttgaggccaggagtttgagaccagcctgggcaacatagcaaggcctcatctctacaaaagaaaaaagaagaacaacaacaacaacaaagttagaggactacatttctggattccaaaacttactacgaagttacaataatcaagacagtgtggtactaccataagatagagcaacagaattgagtccagaaataaacccttatagttagttgatttgtgataagtataaaataattctatagggaaaaaatagtattttcaataagtaatgctaagacaagtgaacatttatgtgcaaaagaatgaggctggatgcttatctcgcactgcatacacaaaaataactcaaaatgggtcaaagagctaaaatcataaaactttagaagaaaacataggggtaacacctcataggcaattgatttagacaatggttttttaggtatgacaccaaaagcataagcaataacataaaaaacagaaatcaagtgaacttcatcaaaatttaaaacttgtactgtatagtatccagaaagtgagaagacaatccatggaatgggagaatatattcacaaagattgtacctgataagaaactagtatccagaatattaaaaagaatgcttacaactcaacaataaaaagacaacccaccgggtgtggtggctcacgcctgtaatcctagcattttgggaggccgaggcaggcagatcacctgagttcaggagttcaagaccagcctggccaacatggcgaaaccctgtctctactaaaaatacaaaaattagccaggcgtgatggtgggtgcctgtaatcccagttactagggaggccgaggcaggagagtcgcttgaactcaggaggtggaggttgcagtgagccgagattgcaccactgcactccaacctgggcgacagagtgagattccatctcagaaaaataaaataaaataacgcagttttaaaatgagaaaggacttgaggccaggcacagtagctaatgtctgtaatgccagcactttgggaagccaaggcagtcagatcacctgaggccaggagttcgagaccagcctggccaacatggtgaaaccctgtctttactaaaaatacaaaaattggctgggcgcggtggctcacgcctgtaatcccagcactttgggaggccaaggcaggcggatcacgaggtcaggagatagagaccatcctggctaacacggtgaaaccctgtctctactaaaaatacaaaaaattagccgggcgtggtggagggcggctgtagtcccagatacttgggaggctgaggcaggagaatggcatgaacccaggaggcggagcttgcagtgagctgagattgcaccactgcactccagcctgggccacagagcgagactccgtctcaaaaaacaatacaaaaattagttgggcatggtggcgagctcctgtaaacccagctactcccaactactagggaggctgaggcaggagaatggcttgaacccagaaggcagaggttacagtgaatcaagataacgccactgcactccaccctgggcgacagagtgagactccgtctcaaaaacaaaaaaataaaaaaaacctcatacactgctggtgggaatataaaatgatgctactactttgaaaagcagtttggcagttcctcaaaaggctaaacatagagttactatatgatgagcactctcacttctaaggtatatgcccagaagaactgaaaacatatatccatataaaaattcatatacgaatattcatagcagcatcatccataatagcaaaaaagtggaaacagtctaaatttcgatcaactgatgaataaactaaatgcggtatatccacacaatagggtattattcagccataaaatgtaatgaagcactggtacactctatagcatagatgaaccttgaaacatgctaagtgaaggaagtcagacacgaaaggccacatgtttatttttataaaatatctagaacaggcaaatcatagagacagaaaatggattattgtttctagaggctgggggaagaggaggattagagtggcagctcactggtatggagtttctaggtagatggaaatgttctggaattagatagtggtgatgattgcacaactctgtaaatatactaaaatccactgcatcatttactttaaaggggcaaattttatggcttgtgaattacatttcaataaaaagaagatgaggaaacctaggatatgtcacaatcccatgccacaaactacttacacttccaatataaaaactatatcaacaatagtttacatcacgttcattgcttgctaaagtaaggtcatgaatgtatcaaaatattttataaaagttaaaatttaggagatccatcatttctcttttcaatccatcactgattcattcaatatatatttatgtgtatgccaggctcttcatcaggtaaagtgtttaggagagatataaagataaaactgatgagaattctgcacttgagctacagcatactttccaagaattacagcatgagatataaaatgaaaagaaggcttggaggagattcacacgaaatagtactgttcaggagagggggcgataattccaatggaagagataactgacttcatggaggatagaaggagatggtatttgaactgcccttgaagtatggttatattttggggatgtggagatgtggggtagggtgatatgctggggttccagatggtccagaaatatacaatcaccagaaccaaagatccagaggtaggagatatgagctgttcaatttggctgagctaacagtgtttggagtgggatcttgaagaagctgaaaatgaagataccaactagacagtcagagaaagacttccaatgtttgactgaactgcaattttattgtgtatgcattgaagaatctttttttttttttttgtattctctaaagatttttaaaatattttaagttctggatacaagtgcaggatgtgcgggtttgttacataggtaaacgtgtcccatggtggtttgctgcacctatcaacctatcacctaggtattaagccccacatgcattagctagttatcctgatgctctccccgctacggcccctgcatcaggccccagtgtgtgttgatctcatccctgtgtccgtgtgttctcattgttcagcttccgcttacaagtgagaacatgtggtgtttggtttcctgctcctctgttagtttgctgaggataatggcttccagcttcatccatgtccctgcaaaggacatgatctcattccttttttaaaaaaaaaaacaaaattatttccataggtgtttggggaacaggtggtatctggttacatgcgtaagtaattaagtggttacttgtgagattctggtgcacccatcacctgagcagtatacactgaacccaatttgtattcttttatccttcacccccctcccaccctttcccctaagtccccaaagtccattgtatccttcttatgcctttgcatcctcatagcttatctcccacttatgagtgagaacatacaatgtttggttttccattcctcagttacttcctttagagtaatagtctccaggttgctgtgaatgtcattaattcattcctttttatggctgagtagtgtttaggtgaggttatttgtaagtaattaatattgagtaaataagattcatccatagtggcaaagccacataacttctaagtatcttaaactatatctaaatggtaccaaaacatgcagtcaattctaaaagctcagctaatgatatttcataatataggaaaatattcacaacatatttttgtgtaaaaaaaagcagacttcaaaatggaatatgcattatgattccaatcatgtaaaagctatacatgaacacatacaaagattaacagatataaacaaatggaagaatgaatggagagatagatgatagacagattgagtggtggtggagaataacagatttaaaaagaaattgtgcctttctatattttcaaaaccatttaaataagtattacctttggagttagaaaatgatatgtattttaaatccataattcaactacttatctatatgatgtcaaactggattaggctgaattatcagcaagtgaataaaacagttccttcatccatggagaaacatccatttatgacattcttggaattcctcttgttagaattctttatgaatttaaaatagaaacatggccagactcaagatttcaatacaaacattactttttcacgttcagtaataaccaattaaaagaattaatgaaaaatctgattcactgtatcaccaaaagctgtaatggctgcactgcacagtattccatggtgtatatgtaccacattttctttatccagtctatctttgatgggcatttgctattgtgtctttgctattgtgaagagtgctgcaatgaacaaaaatgtgcatgtatctttataataaaatggtttatattcctttgggtatatacccagtaatgggattgctgggacaaatagtatttctagttctagatctttgaggaatagccacacacacttccacaacggttgaactaatttacattcccaccaacaatgtaaaagtgttcctacttctccacagcctcgccagcatctgttgttttttgactttttaataatcaccattctgaccggcatgagatggtatctcattgtggttctcctttgcatttctctaatgatcagtaaggttgagcttttttttatatgtttgttggccacataaatgtcttcttttgagaagtgtctgttcatgtcctttgtccactttttgatggggttgtttttttccttgtaaatttgttttaagttccttgtaggttctggatattagacctttgtcagatggatagattgcaaaaatgttctcccattctgtaggttgcctgttcactctaatgatagtttcttttgctgtgcaggagctctttagtttaattagatcccatttgtaatttttgcttttgttgcaattgcttttgatgtttttgtcatgaaacctttgcttgtgcctatgtcttgaatggtattaaatagattttcttctagggtttttatagttttaggttttacattaagtctttaatcttgagttaatttttgtataaggtgtaaggaaggggtcagtttcaattttctgcatatggctagccagttttcccagcaccatttattaaatagggaatcttttccccattgcttgtttttgtcaggtttgtcgatgatcagatggctgtagatgtgtggtcttctttctctggtctctattctgttccattggtctatgtgtctgtttttgtaccagtaccatgccattttggctactgtagccttgcagtatactttgaagttgggtagtgtgatgcttccagctttgttctttttgcttattgttgtcttggttatacgggctcttttttggttccatttgaattttaaagtagtttttttctaattctgtgaagaatgtcaatagtagtttaatgggaatagcaatgaacctataaattactttgggtagtatggccattttcatgatattgattcttcctatccacgagaatggaatgttttttcatttgtgtcctctcttatttccttgagcagtggtttgtagttctccttgaagagatccttcacatcttattagctgtattcctaggtattttattctctttctagcaactgtgaatgggagttcattcatgatttggctctctgcttgtgtattgttggtgtatagaatgcttgtgatttctgcacattgattttgtatcctgagactttgctgaagttgcttatcagcttaaggaacttttgggtggagataatggggttttctagatatagtatcatgtcatctgcaaacacagttttacttcctcttttcctatttgaataccccttatttgtttctcttgcctgattttcttggccagaacttccaatactatgttaaataggagtggtgagacggcatccctgtcttgtgccagttttcaaggggaatgcttccagcttttgcccattcagtatgataatggctgtgggtttgtcataaatggttattattttgagatattttccatcaatacctagtttattgagagtttttaacatgaagcaacgttgaattttattgaaggccttttctgtatctattgagataatcatgtggtttttgtctttagttctgtttatgtgatgaattatgtttcttgatttgcgtatgttgaaccagccttgcatcccagggatgaagccaacattccaaacattttatttattatttatttatttatttatttttgagacagagtctcgcactgtcgcccaggctggagtgcagtggcaagatctcagctcgctgcaagctccacctcccaggttcatgccgttctcttgcctcggcctcccaaatagcagggactacaggcgaccgccacaacgcctggctaattttttgtatttttagtagagacggggttttacatgttagccaggatggtcttgatctcctgacctcgtgatccgcccgccttggcctcccaaagggctgggattataggcgtgagccaccgcacccggcctccaaacattttaatctcataacaatgcatcacttgggttaactaggttgagataaatataaactgtcaattttttttcccctcacataaaagtccagaggtaggtaattagggctgacacagtgattccagtgattctgctccttcgtgccctcatccaacaaggcttcttgctgctcactacccagctacccctacgtgtggcccgtatcttcatggttcaagatggcagctagagctgctaggtagttaagatctctctcacacactttccttctgtcataattaacacagggttttagctcatgaggccaagcatacacattacttcccactggcacccctatgtaatattaaatgcaaagataccctcaggagtcctgtgctcaaaacaagtacaaaataactttttgttgttgtttgtggtgctggtggttttatttatttattttttctgaaacagggtctcactctgtctcccatgctgaagtgcagtggtgtgatcacagctcatcacaaccttgacctctctgggctcaggggatccactcacttcagcctcccaagtagctgggactacaggaacacgccaccacgctcagctaaattttgtctttttttgtagagatggagtcttgctatgttgcccaggctggtctcaaactcctgggctcaagtgatcagtccacctcagcctcccaaagtactcagattataggtatgagccaccatggcatcaaaataacttggaaagtaggaataattgcttgttgttcctgaaaactgtctcttcgacacttttcagactctgttacatgatcatgacaaaatatacacaaatagacatacagatacacatcagttaaaacctcaagaaatagaaaaataaataaatcataaaatatttaaaaagtggtattctgacacactgcccagaggtacccctgttcagcaattttaaaaaattttaaaaatagccctctccccctccctctcttctccctctccccacggtctccctctgatgccgagccgaagctggactgtactgctgccatctcggctcactgcagcctccctgcctgattctcccgcctcggcctgccgcgtgcctgccattgcgggcgccgccacgcctgactggttttcgtatttttttggtggagacagggtttcactgtgttggccgggctggtctccagctcctgactgcgagtgatctgccagcctcggcctcccgaggtgccgggattgcgggcagagtctcgtccactcagtgctcaatgttgcccaggctggagtgcagtggtgtgatctcagctggctacggcctccgcctcccagccgcctgccttggccccccagggtgccgagattacagcttctgcccggccgccaccccgtctgggatgaagtgaggagcgtctctgcccggccgcccatcgtctgagatgtggggagcgcctctgccccgcccccccgtctgggatgtgaggagcttctctgcccggccaccccgtctgagaagtgaggagcccctccgcccgcagctgccccgtctgagaagtgaggagcccctccgcccgacagccaccctgtctgggaagtgaggagcgtctccgcccagcagccaccccgtctgagaagtgaggagcccctccgcctggcagccgccccgtccgggagggaggcgtgggggtcagcccccgcccggccagccgccccgtcggggagggaggtggggggtcagcccccgcccggccagctatcccgtccgggagggaggtggggggcgcgtccgcctggccgccccatctgggaagtgaggagcccctctgcccagccgccaccccgtctgggaggtgtacccaacagctcattgagaacaggccatgatgacgatggcggttttgtggaatagaaaagggggaaaggtggggaaaagatagagaaatcagattgttgctgtgtctgtgtagaaagaagtagacatgggagacttcattttgttctgtactaagaaaaattcttctgccttaggatgctgttgatctatgaccttacccccaaccctgtgctctctgaaacatgtgctgtgtccactcagggttaaatggattaagggcagtgcaagatgtgctttgttaaacagatgcttgaaggcagcatgctccttaagagtcatcaccactccctaatctcaagtacccagggacacaaacactgcggaaggccgcagggtcctctgcctaggaaaaccagagacctttgttcacttgtttatctgctgaccttccctccactattgtcctgtgaccctgccaaatcaccctctgtgagaaacacccaagaatgatcaattaaaaaaaaaaaatttaaaaataataataggccaggtgcagtggctcacacctgtaatcccagcactttgggaggccgaggctggtgaatcacctgaggtcaggagttcaagaccacgctggccaacatggtggaaaccctgtctccactaaaaatacaaaaattagccgggtgtggtggcaggagcctgtaatcccagctactcgggaggctgaggcaggagaatcgcttgaacccagaaggcagaggttgcaatgagccaagatgatgccactgcactccagcctgggcagcagaatgaaactctgtctcaataataataataataataataataataataataataataataataagcaactctaatgatatttcaaacaatggtccccttttaggtcacactatcaaatcagagaaagatatacttgactagctgtaaaatgcaatttgaggtctaggtgaatgaacaagtaacctctaaatcataaggctattgttacaaactgaatgtttgtattccccccagaattcaaaggggagacagtatccccaaagtgacagtatcagaaggtggggcctttgggaggtaattaggtgatgagggtagagccctcatgaatggaatttgtgcccttaaagatatacttgagagtttgcatcctctttttctgccatgtgagaacatcaaaagactgacatctggtaagatctggaagcatgccttaccagacaccagatatgctaccacttagatgttggatttcccagcctccggaactgtgagaaataactgctgtttaagtcacctggtctatggtaatttggtatagttgcccaaatggactgtgatggttaatactgagtatcaacttgattgaatagaaggatgcaaagtgttcccgggtacatctgtgagggtgctgccaaaggagatttaacatttgagtcagtggactgggaaaggcagaccatcctcaatctgggtgggcaccatctaatcagctgccagcactgccagaataaaagcaggcaaaacatggaaagactagactggtgtagtcttctggcctccatctttctctcatgctgaatgcttcctgccctcaaacattggactccaagttcttcagctttgggacttgaattggcttccttgcttgcagatgacctattgtgggacctaaccctgtgatcatgtgagtcaatactccttaataaactcccctttttatatacatgtatcctattagttctgtccctctagagaaacatgactaatacattgagtaagatagttcctgtcctttttttttttttttaaagagatgggatcttgctatattgcccaggttggtatgcagtggctattcgtaggcacaatcacagcatgctatgaccctgaactcctgggttcaaaagatcctcccacctcagcctcccaagtaactgggaatacaggtacccacacccacacccagctaatttttgtatttttactagggacagcgtttaccatgttggccaggctggtctcgaactcctgacctgaagtgatctgccctccttggcctcccaaagtgctgggattacaggtgtgagccactacgcccagccttttggtttcttatgtgtaggagaggataagtttctttctcagagtgtgctgcagccagacataatatttctccttggcagaaactctgctgttccaatcatacatgtagccattgagttcaatgtgaagatccaggagtgggcgttttctttcttgtctcagtttctgggagaggcactgcaggtacagggatggtgagctgtgagactgctccagcagggacatgtccgcagtacacaggctccagaagaagtcagcttctcggtgaactgtgcacagccctcgcttctgagccttgaattccacattcttcatcgctggcccatccacctccaagaggctgctgtcctccagctggccctctgacaccacatagttctgaataaaaaacatctttggcttccctgctagataagggcatgaatctcccatgaacatcctcctgatgtgatgcagggggagccctgagtgagtctgatccacaccatacacactctgggagcctcctcggctcaccaggacacacacaaagctgtcgtagtctcggtgctcgggcatacaggcaaattggccaagaatctgggatataccatgcatactgagatgcaagaatttctggacttcatagcccagggaagtgaaggtgtctcgaagaagctctgtctcattgccaatgcaatcgattatcaggcagattcctaggggcttgctcttcatcttgtatctctcttcaggtatgctctgaggcaaaaaagcttctgattcctgaatggatttcttcactggttcttgttgagcgccaagctgttccttaagtctttgttctttacttctcccattatggagcctgaagttatttgaaggatccttgagactcttttggattgctgcttggagaacattcctgtaacttgtccctgctccttgaacagactgcttgtacttctggatttttgtcttcaggtctattctgtggatgttctttaggcatttttctaataaatccagttgatctggggcaaccagatttagtttctccaactcaaccacaaggtccaagaaactcttctccttgcttatcttgcctcggcccatgtaatccttcatgaggaaaattaatgaggacacatcagatttatccaaatcctcaccaatctctgccatcagcactctatagtccgaaacaaggtgagggttcctgagcaggtgggtctccacagcttttctgtccatcttcaagatacgtttgagcaggtcaaatcgcctcactctgtagagcagttcagccaagtccccgacagacagcttacctctttcccgtaaaatatccagaaggtccctgacattaggtggaaccacatctatagcaacatcccggcacaaaaagagcagcatctccttctcatctgtatcaagtgcttcttcaacctgatggatgacttcagcagacatcctactcttagactagggaagctcacaagggtcttgcagtacagctccgggccagtcaacagaaagccagcaggcagtcaacttcatttctgagggctgacttcatttctttcagaatcctttccagtgggggagttgcccgggcagccgccggctcttcccactggatctccgccgggaccaactcccaccctcgccggacaagctcagacctgctgctccgcaaaaccagaattggaaatgctccagatgggacgaggaacaaggacagaaagtcaaaagcatcaacaggtggcttcgccggagggcgtccgagaacctct

SEQ ID NO: 15631 - RNA, 13510 nt, Homo sapiens
  source 1..13510: mol_type = other RNA
gctgggattacaggcatgagccactgtgcccagcctaaagcgtaataaactttcactgttgctctgaaacttgcctcggtccctccttctgccttatgcccctcagtcaaattctttcttctgaggaggaaagaattgaggttgctgcagatttaccaccagtaacttggataccgtccaccagtaacaacttccgttaagatggcaatacacctcaaatttatttttattttgagacagggtctcactctgttccccaggctggagtacagtggcacaatctcagctcactgaaacctccacctcccgggctcaagtgatcctcccacctcagccttccgagtagctggtactacaggcgcatgctaccatacccagctaatttttgtatttttagtagagacagggttttgccgtgttgcccaaggtggcctcaaattccttggctcaagcgatccaccatcctcagcctcccaaagtcctgggattacaggcatgagccactgcgcccagccaaacttatctttgtatgtttgttataggcaaaagtaccccaaggttaaggctcagcccaagaggtcaagtgggttcaggaaagaattcaagagcatgctgacagaataaagtgaaagcaagttcattaagaaagtaaaggaataaaagaatggctaccccataggaagagtagccctgatgggctgctgactggctatatttatggttgcttcttgactatacgctaaacaagaggtggcttattcatgagttttccaggaaagaagtggggaggtctggaccttttagaccatacagggtaacttctgaaagttgctatggcagttgtaaactatcatggtgctgtagaagtttcttttagcgtgctaatgtattataattaccatagaatgggcagcaaaggtaaccagaggtctcttctgtcaccatcatggttttggctggtttgggttggcctttctaccacatcctgtcttatcagcagggtcttacagggtcttgtggtcttgggaaaccagtcctgccaaactcctctcattcagtgtaatcactatcaaaattccagaggccctttttacataaatttgcaagtgaatcctaacagttatatgaaaatttagggaaaggtaaacccaatacagccctaacaattttgaaaaagaacaggccagttgcagtggctcacccctcagcactttgggaggtggaggtgggaggattgtttgaggccaggagtttgagaccagcctgggcaacatagcaaggcctcatctctacaaaagaaaaaagaagaacaacaacaacaacaaagttagaggactacatttctggattccaaaacttactacgaagttacaataatcaagacagtgtggtactaccataagatagagcaacagaattgagtccagaaataaacccttatagttagttgatttgtgataagtataaaataattctatagggaaaaaatagtattttcaataagtaatgctaagacaagtgaacatttatgtgcaaaagaatgaggctggatgcttatctcgcactgcatacacaaaaataactcaaaatgggtcaaagagctaaaatcataaaactttagaagaaaacataggggtaacacctcataggcaattgatttagacaatggttttttaggtatgacaccaaaagcataagcaataacataaaaaacagaaatcaagtgaacttcatcaaaatttaaaacttgtactgtatagtatccagaaagtgagaagacaatccatggaatgggagaatatattcacaaagattgtacctgataagaaactagtatccagaatattaaaaagaatgcttacaactcaacaataaaaagacaacccaccgggtgtggtggctcacgcctgtaatcctagcattttgggaggccgaggcaggcagatcacctgagttcaggagttcaagaccagcctggccaacatggcgaaaccctgtctctactaaaaatacaaaaattagccaggcgtgatggtgggtgcctgtaatcccagttactagggaggccgaggcaggagagtcgcttgaactcaggaggtggaggttgcagtgagccgagattgcaccactgcactccaacctgggcgacagagtgagattccatctcagaaaaataaaataaaataacgcagttttaaaatgagaaaggacttgaggccaggcacagtagctaatgtctgtaatgccagcactttgggaagccaaggcagtcagatcacctgaggccaggagttcgagaccagcctggccaacatggtgaaaccctgtctttactaaaaatacaaaaattggctgggcgcggtggctcacgcctgtaatcccagcactttgggaggccaaggcaggcggatcacgaggtcaggagatagagaccatcctggctaacacggtgaaaccctgtctctactaaaaatacaaaaaattagccgggcgtggtggagggcggctgtagtcccagatacttgggaggctgaggcaggagaatggcatgaacccaggaggcggagcttgcagtgagctgagattgcaccactgcactccagcctgggccacagagcgagactccgtctcaaaaaacaatacaaaaattagttgggcatggtggcgagctcctgtaaacccagctactcccaactactagggaggctgaggcaggagaatggcttgaacccagaaggcagaggttacagtgaatcaagataacgccactgcactccaccctgggcgacagagtgagactccgtctcaaaaacaaaaaaataaaaaaaacctcatacactgctggtgggaatataaaatgatgctactactttgaaaagcagtttggcagttcctcaaaaggctaaacatagagttactatatgatgagcactctcacttctaaggtatatgcccagaagaactgaaaacatatatccatataaaaattcatatacgaatattcatagcagcatcatccataatagcaaaaaagtggaaacagtctaaatttcgatcaactgatgaataaactaaatgcggtatatccacacaatagggtattattcagccataaaatgtaatgaagcactggtacactctatagcatagatgaaccttgaaacatgctaagtgaaggaagtcagacacgaaaggccacatgtttatttttataaaatatctagaacaggcaaatcatagagacagaaaatggattattgtttctagaggctgggggaagaggaggattagagtggcagctcactggtatggagtttctaggtagatggaaatgttctggaattagatagtggtgatgattgcacaactctgtaaatatactaaaatccactgcatcatttactttaaaggggcaaattttatggcttgtgaattacatttcaataaaaagaagatgaggaaacctaggatatgtcacaatcccatgccacaaactacttacacttccaatataaaaactatatcaacaatagtttacatcacgttcattgcttgctaaagtaaggtcatgaatgtatcaaaatattttataaaagttaaaatttaggagatccatcatttctcttttcaatccatcactgattcattcaatatatatttatgtgtatgccaggctcttcatcaggtaaagtgtttaggagagatataaagataaaactgatgagaattctgcacttgagctacagcatactttccaagaattacagcatgagatataaaatgaaaagaaggcttggaggagattcacacgaaatagtactgttcaggagagggggcgataattccaatggaagagataactgacttcatggaggatagaaggagatggtatttgaactgcccttgaagtatggttatattttggggatgtggagatgtggggtagggtgatatgctggggttccagatggtccagaaatatacaatcaccagaaccaaagatccagaggtaggagatatgagctgttcaatttggctgagctaacagtgtttggagtgggatcttgaagaagctgaaaatgaagataccaactagacagtcagagaaagacttccaatgtttgactgaactgcaattttattgtgtatgcattgaagaatctttttttttttttttgtattctctaaagatttttaaaatattttaagttctggatacaagtgcaggatgtgcgggtttgttacataggtaaacgtgtcccatggtggtttgctgcacctatcaacctatcacctaggtattaagccccacatgcattagctagttatcctgatgctctccccgctacggcccctgcatcaggccccagtgtgtgttgatctcatccctgtgtccgtgtgttctcattgttcagcttccgcttacaagtgagaacatgtggtgtttggtttcctgctcctctgttagtttgctgaggataatggcttccagcttcatccatgtccctgcaaaggacatgatctcattccttttttaaaaaaaaaaacaaaattatttccataggtgtttggggaacaggtggtatctggttacatgcgtaagtaattaagtggttacttgtgagattctggtgcacccatcacctgagcagtatacactgaacccaatttgtattcttttatccttcacccccctcccaccctttcccctaagtccccaaagtccattgtatccttcttatgcctttgcatcctcatagcttatctcccacttatgagtgagaacatacaatgtttggttttccattcctcagttacttcctttagagtaatagtctccaggttgctgtgaatgtcattaattcattcctttttatggctgagtagtgtttaggtgaggttatttgtaagtaattaatattgagtaaataagattcatccatagtggcaaagccacataacttctaagtatcttaaactatatctaaatggtaccaaaacatgcagtcaattctaaaagctcagctaatgatatttcataatataggaaaatattcacaacatatttttgtgtaaaaaaaagcagacttcaaaatggaatatgcattatgattccaatcatgtaaaagctatacatgaacacatacaaagattaacagatataaacaaatggaagaatgaatggagagatagatgatagacagattgagtggtggtggagaataacagatttaaaaagaaattgtgcctttctatattttcaaaaccatttaaataagtattacctttggagttagaaaatgatatgtattttaaatccataattcaactacttatctatatgatgtcaaactggattaggctgaattatcagcaagtgaataaaacagttccttcatccatggagaaacatccatttatgacattcttggaattcctcttgttagaattctttatgaatttaaaatagaaacatggccagactcaagatttcaatacaaacattactttttcacgttcagtaataaccaattaaaagaattaatgaaaaatctgattcactgtatcaccaaaagctgtaatggctgcactgcacagtattccatggtgtatatgtaccacattttctttatccagtctatctttgatgggcatttgctattgtgtctttgctattgtgaagagtgctgcaatgaacaaaaatgtgcatgtatctttataataaaatggtttatattcctttgggtatatacccagtaatgggattgctgggacaaatagtatttctagttctagatctttgaggaatagccacacacacttccacaacggttgaactaatttacattcccaccaacaatgtaaaagtgttcctacttctccacagcctcgccagcatctgttgttttttgactttttaataatcaccattctgaccggcatgagatggtatctcattgtggttctcctttgcatttctctaatgatcagtaaggttgagcttttttttatatgtttgttggccacataaatgtcttcttttgagaagtgtctgttcatgtcctttgtccactttttgatggggttgtttttttccttgtaaatttgttttaagttccttgtaggttctggatattagacctttgtcagatggatagattgcaaaaatgttctcccattctgtaggttgcctgttcactctaatgatagtttcttttgctgtgcaggagctctttagtttaattagatcccatttgtaatttttgcttttgttgcaattgcttttgatgtttttgtcatgaaacctttgcttgtgcctatgtcttgaatggtattaaatagattttcttctagggtttttatagttttaggttttacattaagtctttaatcttgagttaatttttgtataaggtgtaaggaaggggtcagtttcaattttctgcatatggctagccagttttcccagcaccatttattaaatagggaatcttttccccattgcttgtttttgtcaggtttgtcgatgatcagatggctgtagatgtgtggtcttctttctctggtctctattctgttccattggtctatgtgtctgtttttgtaccagtaccatgccattttggctactgtagccttgcagtatactttgaagttgggtagtgtgatgcttccagctttgttctttttgcttattgttgtcttggttatacgggctcttttttggttccatttgaattttaaagtagtttttttctaattctgtgaagaatgtcaatagtagtttaatgggaatagcaatgaacctataaattactttgggtagtatggccattttcatgatattgattcttcctatccacgagaatggaatgttttttcatttgtgtcctctcttatttccttgagcagtggtttgtagttctccttgaagagatccttcacatcttattagctgtattcctaggtattttattctctttctagcaactgtgaatgggagttcattcatgatttggctctctgcttgtgtattgttggtgtatagaatgcttgtgatttctgcacattgattttgtatcctgagactttgctgaagttgcttatcagcttaaggaacttttgggtggagataatggggttttctagatatagtatcatgtcatctgcaaacacagttttacttcctcttttcctatttgaataccccttatttgtttctcttgcctgattttcttggccagaacttccaatactatgttaaataggagtggtgagacggcatccctgtcttgtgccagttttcaaggggaatgcttccagcttttgcccattcagtatgataatggctgtgggtttgtcataaatggttattattttgagatattttccatcaatacctagtttattgagagtttttaacatgaagcaacgttgaattttattgaaggccttttctgtatctattgagataatcatgtggtttttgtctttagttctgtttatgtgatgaattatgtttcttgatttgcgtatgttgaaccagccttgcatcccagggatgaagccaacattccaaacattttatttattatttatttatttatttatttttgagacagagtctcgcactgtcgcccaggctggagtgcagtggcaagatctcagctcgctgcaagctccacctcccaggttcatgccgttctcttgcctcggcctcccaaatagcagggactacaggcgaccgccacaacgcctggctaattttttgtatttttagtagagacggggttttacatgttagccaggatggtcttgatctcctgacctcgtgatccgcccgccttggcctcccaaagggctgggattataggcgtgagccaccgcacccggcctccaaacattttaatctcataacaatgcatcacttgggttaactaggttgagataaatataaactgtcaattttttttcccctcacataaaagtccagaggtaggtaattagggctgacacagtgattccagtgattctgctccttcgtgccctcatccaacaaggcttcttgctgctcactacccagctacccctacgtgtggcccgtatcttcatggttcaagatggcagctagagctgctaggtagttaagatctctctcacacactttccttctgtcataattaacacagggttttagctcatgaggccaagcatacacattacttcccactggcacccctatgtaatattaaatgcaaagataccctcaggagtcctgtgctcaaaacaagtacaaaataactttttgttgttgtttgtggtgctggtggttttatttatttattttttctgaaacagggtctcactctgtctcccatgctgaagtgcagtggtgtgatcacagctcatcacaaccttgacctctctgggctcaggggatccactcacttcagcctcccaagtagctgggactacaggaacacgccaccacgctcagctaaattttgtctttttttgtagagatggagtcttgctatgttgcccaggctggtctcaaactcctgggctcaagtgatcagtccacctcagcctcccaaagtactcagattataggtatgagccaccatggcatcaaaataacttggaaagtaggaataattgcttgttgttcctgaaaactgtctcttcgacacttttcagactctgttacatgatcatgacaaaatatacacaaatagacatacagatacacatcagttaaaacctcaagaaatagaaaaataaataaatcataaaatatttaaaaagtggtattctgacacactgcccagaggtacccctgttcagcaattttaaaaaattttaaaaatagccctctccccctccctctcttctccctctccccacggtctccctctgatgccgagccgaagctggactgtactgctgccatctcggctcactgcagcctccctgcctgattctcccgcctcggcctgccgcgtgcctgccattgcgggcgccgccacgcctgactggttttcgtatttttttggtggagacagggtttcactgtgttggccgggctggtctccagctcctgactgcgagtgatctgccagcctcggcctcccgaggtgccgggattgcgggcagagtctcgtccactcagtgctcaatgttgcccaggctggagtgcagtggtgtgatctcagctggctacggcctccgcctcccagccgcctgccttggccccccagggtgccgagattacagcttctgcccggccgccaccccgtctgggatgaagtgaggagcgtctctgcccggccgcccatcgtctgagatgtggggagcgcctctgccccgcccccccgtctgggatgtgaggagcttctctgcccggccaccccgtctgagaagtgaggagcccctccgcccgcagctgccccgtctgagaagtgaggagcccctccgcccgacagccaccctgtctgggaagtgaggagcgtctccgcccagcagccaccccgtctgagaagtgaggagcccctccgcctggcagccgccccgtccgggagggaggcgtgggggtcagcccccgcccggccagccgccccgtcggggagggaggtggggggtcagcccccgcccggccagctatcccgtccgggagggaggtggggggcgcgtccgcctggccgccccatctgggaagtgaggagcccctctgcccagccgccaccccgtctgggaggtgtacccaacagctcattgagaacaggccatgatgacgatggcggttttgtggaatagaaaagggggaaaggtggggaaaagatagagaaatcagattgttgctgtgtctgtgtagaaagaagtagacatgggagacttcattttgttctgtactaagaaaaattcttctgccttaggatgctgttgatctatgaccttacccccaaccctgtgctctctgaaacatgtgctgtgtccactcagggttaaatggattaagggcagtgcaagatgtgctttgttaaacagatgcttgaaggcagcatgctccttaagagtcatcaccactccctaatctcaagtacccagggacacaaacactgcggaaggccgcagggtcctctgcctaggaaaaccagagacctttgttcacttgtttatctgctgaccttccctccactattgtcctgtgaccctgccaaatcaccctctgtgagaaacacccaagaatgatcaattaaaaaaaaaaaatttaaaaataataataggccaggtgcagtggctcacacctgtaatcccagcactttgggaggccgaggctggtgaatcacctgaggtcaggagttcaagaccacgctggccaacatggtggaaaccctgtctccactaaaaatacaaaaattagccgggtgtggtggcaggagcctgtaatcccagctactcgggaggctgaggcaggagaatcgcttgaacccagaaggcagaggttgcaatgagccaagatgatgccactgcactccagcctgggcagcagaatgaaactctgtctcaataataataataataataataataataataataataataataataagcaactctaatgatatttcaaacaatggtccccttttaggtcacactatcaaatcagagaaagatatacttgactagctgtaaaatgcaatttgaggtctaggtgaatgaacaagtaacctctaaatcataaggctattgttacaaactgaatgtttgtattccccccagaattcaaaggggagacagtatccccaaagtgacagtatcagaaggtggggcctttgggaggtaattaggtgatgagggtagagccctcatgaatggaatttgtgcccttaaagatatacttgagagtttgcatcctctttttctgccatgtgagaacatcaaaagactgacatctggtaagatctggaagcatgccttaccagacaccagatatgctaccacttagatgttggatttcccagcctccggaactgtgagaaataactgctgtttaagtcacctggtctatggtaatttggtatagttgcccaaatggactgtgatggttaatactgagtatcaacttgattgaatagaaggatgcaaagtgttcccgggtacatctgtgagggtgctgccaaaggagatttaacatttgagtcagtggactgggaaaggcagaccatcctcaatctgggtgggcaccatctaatcagctgccagcactgccagaataaaagcaggcaaaacatggaaagactagactggtgtagtcttctggcctccatctttctctcatgctgaatgcttcctgccctcaaacattggactccaagttcttcagctttgggacttgaattggcttccttgcttgcagatgacctattgtgggacctaaccctgtgatcatgtgagtcaatactccttaataaactcccctttttatatacatgtatcctattagttctgtccctctagagaaacatgactaatacattgagtaagatagttcctgtcctttttttttttttttaaagagatgggatcttgctatattgcccaggttggtatgcagtggctattcgtaggcacaatcacagcatgctatgaccctgaactcctgggttcaaaagatcctcccacctcagcctcccaagtaactgggaatacaggtacccacacccacacccagctaatttttgtatttttactagggacagcgtttaccatgttggccaggctggtctcgaactcctgacctgaagtgatctgccctccttggcctcccaaagtgctgggattacaggtgtgagccactacgcccagccttttggtttcttatgtgtaggagaggataagtttctttctcagagtgtgctgcagccagacataatatttctccttggcagaaactctgctgttccaatcatacatgtagccattgagttcaatgtgaagatccaggagtgggcgttttctttcttgtctcagtttctgggagaggcactgcaggtacagggatggtgagctgtgagactgctccagcagggacatgtccgcagtacacaggctccagaagaagtcagcttctcggtgaactgtgcacagccctcgcttctgagccttgaattccacattcttcatcgctggcccatccacctccaagaggctgctgtcctccagctggccctctgacaccacatagttctgaataaaaaacatctttggcttccctgctagataagggcatgaatctcccatgaacatcctcctgatgtgatgcagggggagccctgagtgagtctgatccacaccatacacactctgggagcctcctcggctcaccaggacacacacaaagctgtcgtagtctcggtgctcgggcatacaggcaaattggccaagaatctgggatataccatgcatactgagatgcaagaatttctggacttcatagcccagggaagtgaaggtgtctcgaagaagctctgtctcattgccaatgcaatcgattatcaggcagattcctaggggcttgctcttcatcttgtatctctcttcaggtatgctctgaggcaaaaaagcttctgattcctgaatggatttcttcactggttcttgttgagcgccaagctgttccttaagtctttgttctttacttctcccattatggagcctgaagttatttgaaggatccttgagactcttttggattgctgcttggagaacattcctgtaacttgtccctgctccttgaacagactgcttgtacttctggatttttgtcttcaggtctattctgtggatgttctttaggcatttttctaataaatccagttgatctggggcaaccagatttagtttctccaactcaaccacaaggtccaagaaactcttctccttgcttatcttgcctcggcccatgtaatccttcatgaggaaaattaatgaggacacatcagatttatccaaatcctcaccaatctctgccatcagcactctctttcccgtaaaatatccagaaggtccctgacattaggtggaaccacatctatagcaacatcccggcacaaaaagagcagcatctccttctcatctgtatcaagtgcttcttcaacctgatggatgacttcagcagacatcctactcttagactagggaagctcacaagggtcttgcagtacagctccgggccagtcaacagaaagccagcaggcagtcaacttcatttctgagggctgacttcatttctttcagaatcctttccagtgggggagttgcccgggcagccgccggctcttcccactggatctccgccgggaccaactcccaccctcgccggacaagctcagacctgctgctccgcaaaaccagaattggaaatgctccagatgggacgaggaacaaggacagaaagtcaaaagcatcaacaggtggcttcgccggagggcgtccgagaacctct

SEQ ID NO: 15632 - RNA, 13231 nt, Homo sapiens
  source 1..13231: mol_type = other RNA
gctgggattacaggcatgagccactgtgcccagcctaaagcgtaataaactttcactgttgctctgaaacttgcctcggtccctccttctgccttatgcccctcagtcaaattctttcttctgaggaggaaagaattgaggttgctgcagatttaccaccagtaacttggataccgtccaccagtaacaacttccgttaagatggcaatacacctcaaatttatttttattttgagacagggtctcactctgttccccaggctggagtacagtggcacaatctcagctcactgaaacctccacctcccgggctcaagtgatcctcccacctcagccttccgagtagctggtactacaggcgcatgctaccatacccagctaatttttgtatttttagtagagacagggttttgccgtgttgcccaaggtggcctcaaattccttggctcaagcgatccaccatcctcagcctcccaaagtcctgggattacaggcatgagccactgcgcccagccaaacttatctttgtatgtttgttataggcaaaagtaccccaaggttaaggctcagcccaagaggtcaagtgggttcaggaaagaattcaagagcatgctgacagaataaagtgaaagcaagttcattaagaaagtaaaggaataaaagaatggctaccccataggaagagtagccctgatgggctgctgactggctatatttatggttgcttcttgactatacgctaaacaagaggtggcttattcatgagttttccaggaaagaagtggggaggtctggaccttttagaccatacagggtaacttctgaaagttgctatggcagttgtaaactatcatggtgctgtagaagtttcttttagcgtgctaatgtattataattaccatagaatgggcagcaaaggtaaccagaggtctcttctgtcaccatcatggttttggctggtttgggttggcctttctaccacatcctgtcttatcagcagggtcttacagggtcttgtggtcttgggaaaccagtcctgccaaactcctctcattcagtgtaatcactatcaaaattccagaggccctttttacataaatttgcaagtgaatcctaacagttatatgaaaatttagggaaaggtaaacccaatacagccctaacaattttgaaaaagaacaggccagttgcagtggctcacccctcagcactttgggaggtggaggtgggaggattgtttgaggccaggagtttgagaccagcctgggcaacatagcaaggcctcatctctacaaaagaaaaaagaagaacaacaacaacaacaaagttagaggactacatttctggattccaaaacttactacgaagttacaataatcaagacagtgtggtactaccataagatagagcaacagaattgagtccagaaataaacccttatagttagttgatttgtgataagtataaaataattctatagggaaaaaatagtattttcaataagtaatgctaagacaagtgaacatttatgtgcaaaagaatgaggctggatgcttatctcgcactgcatacacaaaaataactcaaaatgggtcaaagagctaaaatcataaaactttagaagaaaacataggggtaacacctcataggcaattgatttagacaatggttttttaggtatgacaccaaaagcataagcaataacataaaaaacagaaatcaagtgaacttcatcaaaatttaaaacttgtactgtatagtatccagaaagtgagaagacaatccatggaatgggagaatatattcacaaagattgtacctgataagaaactagtatccagaatattaaaaagaatgcttacaactcaacaataaaaagacaacccaccgggtgtggtggctcacgcctgtaatcctagcattttgggaggccgaggcaggcagatcacctgagttcaggagttcaagaccagcctggccaacatggcgaaaccctgtctctactaaaaatacaaaaattagccaggcgtgatggtgggtgcctgtaatcccagttactagggaggccgaggcaggagagtcgcttgaactcaggaggtggaggttgcagtgagccgagattgcaccactgcactccaacctgggcgacagagtgagattccatctcagaaaaataaaataaaataacgcagttttaaaatgagaaaggacttgaggccaggcacagtagctaatgtctgtaatgccagcactttgggaagccaaggcagtcagatcacctgaggccaggagttcgagaccagcctggccaacatggtgaaaccctgtctttactaaaaatacaaaaattggctgggcgcggtggctcacgcctgtaatcccagcactttgggaggccaaggcaggcggatcacgaggtcaggagatagagaccatcctggctaacacggtgaaaccctgtctctactaaaaatacaaaaaattagccgggcgtggtggagggcggctgtagtcccagatacttgggaggctgaggcaggagaatggcatgaacccaggaggcggagcttgcagtgagctgagattgcaccactgcactccagcctgggccacagagcgagactccgtctcaaaaaacaatacaaaaattagttgggcatggtggcgagctcctgtaaacccagctactcccaactactagggaggctgaggcaggagaatggcttgaacccagaaggcagaggttacagtgaatcaagataacgccactgcactccaccctgggcgacagagtgagactccgtctcaaaaacaaaaaaataaaaaaaacctcatacactgctggtgggaatataaaatgatgctactactttgaaaagcagtttggcagttcctcaaaaggctaaacatagagttactatatgatgagcactctcacttctaaggtatatgcccagaagaactgaaaacatatatccatataaaaattcatatacgaatattcatagcagcatcatccataatagcaaaaaagtggaaacagtctaaatttcgatcaactgatgaataaactaaatgcggtatatccacacaatagggtattattcagccataaaatgtaatgaagcactggtacactctatagcatagatgaaccttgaaacatgctaagtgaaggaagtcagacacgaaaggccacatgtttatttttataaaatatctagaacaggcaaatcatagagacagaaaatggattattgtttctagaggctgggggaagaggaggattagagtggcagctcactggtatggagtttctaggtagatggaaatgttctggaattagatagtggtgatgattgcacaactctgtaaatatactaaaatccactgcatcatttactttaaaggggcaaattttatggcttgtgaattacatttcaataaaaagaagatgaggaaacctaggatatgtcacaatcccatgccacaaactacttacacttccaatataaaaactatatcaacaatagtttacatcacgttcattgcttgctaaagtaaggtcatgaatgtatcaaaatattttataaaagttaaaatttaggagatccatcatttctcttttcaatccatcactgattcattcaatatatatttatgtgtatgccaggctcttcatcaggtaaagtgtttaggagagatataaagataaaactgatgagaattctgcacttgagctacagcatactttccaagaattacagcatgagatataaaatgaaaagaaggcttggaggagattcacacgaaatagtactgttcaggagagggggcgataattccaatggaagagataactgacttcatggaggatagaaggagatggtatttgaactgcccttgaagtatggttatattttggggatgtggagatgtggggtagggtgatatgctggggttccagatggtccagaaatatacaatcaccagaaccaaagatccagaggtaggagatatgagctgttcaatttggctgagctaacagtgtttggagtgggatcttgaagaagctgaaaatgaagataccaactagacagtcagagaaagacttccaatgtttgactgaactgcaattttattgtgtatgcattgaagaatctttttttttttttttgtattctctaaagatttttaaaatattttaagttctggatacaagtgcaggatgtgcgggtttgttacataggtaaacgtgtcccatggtggtttgctgcacctatcaacctatcacctaggtattaagccccacatgcattagctagttatcctgatgctctccccgctacggcccctgcatcaggccccagtgtgtgttgatctcatccctgtgtccgtgtgttctcattgttcagcttccgcttacaagtgagaacatgtggtgtttggtttcctgctcctctgttagtttgctgaggataatggcttccagcttcatccatgtccctgcaaaggacatgatctcattccttttttaaaaaaaaaaacaaaattatttccataggtgtttggggaacaggtggtatctggttacatgcgtaagtaattaagtggttacttgtgagattctggtgcacccatcacctgagcagtatacactgaacccaatttgtattcttttatccttcacccccctcccaccctttcccctaagtccccaaagtccattgtatccttcttatgcctttgcatcctcatagcttatctcccacttatgagtgagaacatacaatgtttggttttccattcctcagttacttcctttagagtaatagtctccaggttgctgtgaatgtcattaattcattcctttttatggctgagtagtgtttaggtgaggttatttgtaagtaattaatattgagtaaataagattcatccatagtggcaaagccacataacttctaagtatcttaaactatatctaaatggtaccaaaacatgcagtcaattctaaaagctcagctaatgatatttcataatataggaaaatattcacaacatatttttgtgtaaaaaaaagcagacttcaaaatggaatatgcattatgattccaatcatgtaaaagctatacatgaacacatacaaagattaacagatataaacaaatggaagaatgaatggagagatagatgatagacagattgagtggtggtggagaataacagatttaaaaagaaattgtgcctttctatattttcaaaaccatttaaataagtattacctttggagttagaaaatgatatgtattttaaatccataattcaactacttatctatatgatgtcaaactggattaggctgaattatcagcaagtgaataaaacagttccttcatccatggagaaacatccatttatgacattcttggaattcctcttgttagaattctttatgaatttaaaatagaaacatggccagactcaagatttcaatacaaacattactttttcacgttcagtaataaccaattaaaagaattaatgaaaaatctgattcactgtatcaccaaaagctgtaatggctgcactgcacagtattccatggtgtatatgtaccacattttctttatccagtctatctttgatgggcatttgctattgtgtctttgctattgtgaagagtgctgcaatgaacaaaaatgtgcatgtatctttataataaaatggtttatattcctttgggtatatacccagtaatgggattgctgggacaaatagtatttctagttctagatctttgaggaatagccacacacacttccacaacggttgaactaatttacattcccaccaacaatgtaaaagtgttcctacttctccacagcctcgccagcatctgttgttttttgactttttaataatcaccattctgaccggcatgagatggtatctcattgtggttctcctttgcatttctctaatgatcagtaaggttgagcttttttttatatgtttgttggccacataaatgtcttcttttgagaagtgtctgttcatgtcctttgtccactttttgatggggttgtttttttccttgtaaatttgttttaagttccttgtaggttctggatattagacctttgtcagatggatagattgcaaaaatgttctcccattctgtaggttgcctgttcactctaatgatagtttcttttgctgtgcaggagctctttagtttaattagatcccatttgtaatttttgcttttgttgcaattgcttttgatgtttttgtcatgaaacctttgcttgtgcctatgtcttgaatggtattaaatagattttcttctagggtttttatagttttaggttttacattaagtctttaatcttgagttaatttttgtataaggtgtaaggaaggggtcagtttcaattttctgcatatggctagccagttttcccagcaccatttattaaatagggaatcttttccccattgcttgtttttgtcaggtttgtcgatgatcagatggctgtagatgtgtggtcttctttctctggtctctattctgttccattggtctatgtgtctgtttttgtaccagtaccatgccattttggctactgtagccttgcagtatactttgaagttgggtagtgtgatgcttccagctttgttctttttgcttattgttgtcttggttatacgggctcttttttggttccatttgaattttaaagtagtttttttctaattctgtgaagaatgtcaatagtagtttaatgggaatagcaatgaacctataaattactttgggtagtatggccattttcatgatattgattcttcctatccacgagaatggaatgttttttcatttgtgtcctctcttatttccttgagcagtggtttgtagttctccttgaagagatccttcacatcttattagctgtattcctaggtattttattctctttctagcaactgtgaatgggagttcattcatgatttggctctctgcttgtgtattgttggtgtatagaatgcttgtgatttctgcacattgattttgtatcctgagactttgctgaagttgcttatcagcttaaggaacttttgggtggagataatggggttttctagatatagtatcatgtcatctgcaaacacagttttacttcctcttttcctatttgaataccccttatttgtttctcttgcctgattttcttggccagaacttccaatactatgttaaataggagtggtgagacggcatccctgtcttgtgccagttttcaaggggaatgcttccagcttttgcccattcagtatgataatggctgtgggtttgtcataaatggttattattttgagatattttccatcaatacctagtttattgagagtttttaacatgaagcaacgttgaattttattgaaggccttttctgtatctattgagataatcatgtggtttttgtctttagttctgtttatgtgatgaattatgtttcttgatttgcgtatgttgaaccagccttgcatcccagggatgaagccaacattccaaacattttatttattatttatttatttatttatttttgagacagagtctcgcactgtcgcccaggctggagtgcagtggcaagatctcagctcgctgcaagctccacctcccaggttcatgccgttctcttgcctcggcctcccaaatagcagggactacaggcgaccgccacaacgcctggctaattttttgtatttttagtagagacggggttttacatgttagccaggatggtcttgatctcctgacctcgtgatccgcccgccttggcctcccaaagggctgggattataggcgtgagccaccgcacccggcctccaaacattttaatctcataacaatgcatcacttgggttaactaggttgagataaatataaactgtcaattttttttcccctcacataaaagtccagaggtaggtaattagggctgacacagtgattccagtgattctgctccttcgtgccctcatccaacaaggcttcttgctgctcactacccagctacccctacgtgtggcccgtatcttcatggttcaagatggcagctagagctgctaggtagttaagatctctctcacacactttccttctgtcataattaacacagggttttagctcatgaggccaagcatacacattacttcccactggcacccctatgtaatattaaatgcaaagataccctcaggagtcctgtgctcaaaacaagtacaaaataactttttgttgttgtttgtggtgctggtggttttatttatttattttttctgaaacagggtctcactctgtctcccatgctgaagtgcagtggtgtgatcacagctcatcacaaccttgacctctctgggctcaggggatccactcacttcagcctcccaagtagctgggactacaggaacacgccaccacgctcagctaaattttgtctttttttgtagagatggagtcttgctatgttgcccaggctggtctcaaactcctgggctcaagtgatcagtccacctcagcctcccaaagtactcagattataggtatgagccaccatggcatcaaaataacttggaaagtaggaataattgcttgttgttcctgaaaactgtctcttcgacacttttcagactctgttacatgatcatgacaaaatatacacaaatagacatacagatacacatcagttaaaacctcaagaaatagaaaaataaataaatcataaaatatttaaaaagtggtattctgacacactgcccagaggtacccctgttcagcaattttaaaaaattttaaaaatagccctctccccctccctctcttctccctctccccacggtctccctctgatgccgagccgaagctggactgtactgctgccatctcggctcactgcagcctccctgcctgattctcccgcctcggcctgccgcgtgcctgccattgcgggcgccgccacgcctgactggttttcgtatttttttggtggagacagggtttcactgtgttggccgggctggtctccagctcctgactgcgagtgatctgccagcctcggcctcccgaggtgccgggattgcgggcagagtctcgtccactcagtgctcaatgttgcccaggctggagtgcagtggtgtgatctcagctggctacggcctccgcctcccagccgcctgccttggccccccagggtgccgagattacagcttctgcccggccgccaccccgtctgggatgaagtgaggagcgtctctgcccggccgcccatcgtctgagatgtggggagcgcctctgccccgcccccccgtctgggatgtgaggagcttctctgcccggccaccccgtctgagaagtgaggagcccctccgcccgcagctgccccgtctgagaagtgaggagcccctccgcccgacagccaccctgtctgggaagtgaggagcgtctccgcccagcagccaccccgtctgagaagtgaggagcccctccgcctggcagccgccccgtccgggagggaggcgtgggggtcagcccccgcccggccagccgccccgtcggggagggaggtggggggtcagcccccgcccggccagctatcccgtccgggagggaggtggggggcgcgtccgcctggccgccccatctgggaagtgaggagcccctctgcccagccgccaccccgtctgggaggtgtacccaacagctcattgagaacaggccatgatgacgatggcggttttgtggaatagaaaagggggaaaggtggggaaaagatagagaaatcagattgttgctgtgtctgtgtagaaagaagtagacatgggagacttcattttgttctgtactaagaaaaattcttctgccttaggatgctgttgatctatgaccttacccccaaccctgtgctctctgaaacatgtgctgtgtccactcagggttaaatggattaagggcagtgcaagatgtgctttgttaaacagatgcttgaaggcagcatgctccttaagagtcatcaccactccctaatctcaagtacccagggacacaaacactgcggaaggccgcagggtcctctgcctaggaaaaccagagacctttgttcacttgtttatctgctgaccttccctccactattgtcctgtgaccctgccaaatcaccctctgtgagaaacacccaagaatgatcaattaaaaaaaaaaaatttaaaaataataataggccaggtgcagtggctcacacctgtaatcccagcactttgggaggccgaggctggtgaatcacctgaggtcaggagttcaagaccacgctggccaacatggtggaaaccctgtctccactaaaaatacaaaaattagccgggtgtggtggcaggagcctgtaatcccagctactcgggaggctgaggcaggagaatcgcttgaacccagaaggcagaggttgcaatgagccaagatgatgccactgcactccagcctgggcagcagaatgaaactctgtctcaataataataataataataataataataataataataataataataagcaactctaatgatatttcaaacaatggtccccttttaggtcacactatcaaatcagagaaagatatacttgactagctgtaaaatgcaatttgaggtctaggtgaatgaacaagtaacctctaaatcataaggctattgttacaaactgaatgtttgtattccccccagaattcaaaggggagacagtatccccaaagtgacagtatcagaaggtggggcctttgggaggtaattaggtgatgagggtagagccctcatgaatggaatttgtgcccttaaagatatacttgagagtttgcatcctctttttctgccatgtgagaacatcaaaagactgacatctggtaagatctggaagcatgccttaccagacaccagatatgctaccacttagatgttggatttcccagcctccggaactgtgagaaataactgctgtttaagtcacctggtctatggtaatttggtatagttgcccaaatggactgtgatggttaatactgagtatcaacttgattgaatagaaggatgcaaagtgttcccgggtacatctgtgagggtgctgccaaaggagatttaacatttgagtcagtggactgggaaaggcagaccatcctcaatctgggtgggcaccatctaatcagctgccagcactgccagaataaaagcaggcaaaacatggaaagactagactggtgtagtcttctggcctccatctttctctcatgctgaatgcttcctgccctcaaacattggactccaagttcttcagctttgggacttgaattggcttccttgcttgcagatgacctattgtgggacctaaccctgtgatcatgtgagtcaatactccttaataaactcccctttttatatacatgtatcctattagttctgtccctctagagaaacatgactaatacattgagtaagatagttcctgtcctttttttttttttttaaagagatgggatcttgctatattgcccaggttggtatgcagtggctattcgtaggcacaatcacagcatgctatgaccctgaactcctgggttcaaaagatcctcccacctcagcctcccaagtaactgggaatacaggtacccacacccacacccagctaatttttgtatttttactagggacagcgtttaccatgttggccaggctggtctcgaactcctgacctgaagtgatctgccctccttggcctcccaaagtgctgggattacaggtgtgagccactacgcccagccttttggtttcttatgtgtaggagaggataagtttctttctcagagtgtgctgcagccagacataatatttctccttggcagaaactctgctgttccaatcatacatgtagccattgagttcaatgtgaagatccaggagtgggcgttttctttcttgtctcagtttctgggagaggcactgcaggtacagggatggtgagctgtgagactgctccagcagggacatgtccgcagtacacaggctccagaagaagtcagcttctcggtgaactgtgcacagccctcgcttctgagccttgaattccacattcttcatcgctggcccatccacctccaagaggctgctgtcctccagctggccctctgacaccacatagttctgaataaaaaacatctttggcttccctgctagataagggcatgaatctcccatgaacatcctcctgatgtgatgcagggggagccctgagtgagtctgatccacaccatacacactctgggagcctcctcggctcaccaggacacacacaaagctgtcgtagtctcggtgctcgggcatacaggcaaattggccaagaatctgggatataccatgcatactgagatgcaagaatttctggacttcatagcccagggaagtgaaggtgtctcgaagaagctctgtctcattgccaatgcaatcgattatcaggcagattcctaggggcttgctcttcatcttgtatctctcttcaggtatgctctgaggcaaaaaagcttctgattcctgaatggatttcttcactggttcttgttgagcgccaagctgttccttaagtctttgttctttacttctcccattatggagcctgaagttatttgaaggatccttgagactcttttggattgctgcttggagaacattcctgtaacttgtccctgctccttgaacagactgcttgtacttctggatttttgtcttcaggtctattctgtggatgttctttaggcatttttctaataaatccagttgatctggggcaaccagatttagtttctccaactcaaccacaaggtccaagaaactcttctccttgcttatcttgcctcggcccatgtaatccttcatgaggaaaattaatgaggacacatcagatttatccaaatcctcaccaatctctgccatcagcactgcccgggcagccgccggctcttcccactggatctccgccgggaccaactcccaccctcgccggacaagctcagacctgctgctccgcaaaaccagaattggaaatgctccagatgggacgaggaacaaggacagaaagtcaaaagcatcaacaggtggcttcgccggagggcgtccgagaacctct

SEQ ID NO: 15633 - RNA, 7281 nt, Homo sapiens
  source 1..7281: mol_type = other RNA
gctgggattacaggcatgagccactgtgcccagcctaatttgattattttgcttatctgtcctaagtttcctcacctctgaaatgagaatatcattaatacttatttcaggagctgatgattcagttgttacacataaagcattaataactgtgattcttactctaaatgtgattgatataaaatatatatgcaaagataaatcacttattaaagaatatatatcagttttttaaaatggaaacaaatctaaggggagtatattaaatggcagctgtcattgcaaaagttgcacaaatatcatgttttgctgtaagatcctctggctcagaaaagaaataccagccacagtaggaagttgaattgcctccagggattcaatgagagaaattatctcctttgcataaatgataattaatatcttggggactctcttattaactgtattttcatttacttctccagatgctggttaacctccacacgcttgattttcaagcatctgatctttgataacttccatattaagagacttcatttcaccatctagtatccctgtactttaattgaactaaagatttacaaggacactccattttcctatttacagagaacctagtctgtacctgccattgttttacatacattttcatgtcacaaaattttatttctaaacaacaccctcatttatgtattttctaagtgttcactggagtaacacagagaagaaatgcagtaaacatataatttggattaaaatgtatggaaggaaaaaatccttaaagtaaaaatcatatacaaaaacaaaaagtcattttactactattggctcatggctgtaatcctagcactttgggaagctgaggcaggaggaatgcttgaggccaagagttcaagaccaacctggccaacatagcgagaccccacgtctaaaaagaaaaagaaaaaaaaaaagaaaagaagctatggagaatatgttacacaataccataaactgaacaagacatgaatataacacagcctttggaaaaatgccctttggctaaaattgcttgatcatattatgtaataaacttttccacaaattcatttgcattgaactactgtaaaaatattttaggcaatttaaacagcatttcacaaatattttcaagaatgacgttgtgtaatgggccctatgggttcagcagaaaggaagagtattatctactattatgaagaaagcggaggtcttccctaacaaagaagttagaaatttcttttgtttttttgagagtctcactctattgcccaggctggagtgcagtggtgagatctcagctcactgcaacctccgtctcccgggttcaagtgattctcctgcctcagcctccctggtagctaggactacaggagtgcgccaccacacctggctaatttttgtatttttagtagagatggggtttcaccatgttggccaggctcgtcttgagctcctgacctaaggtgatccacctgcctcgggctcccaaagtgctgggattacaggcatgagcctgtaatttctggccatgcctggccagaaatcagaagttgcaagagtaaatattcagtgttgtactacagtcagtttccattttgtgatttttgtcttataccaccatttatacctctgcactccctcttcttattctgcccatctggccaagctgataatgtccgtgttccctcctttggcactagatggaagttcaaatcacgtgtgggatcctcaccccaacccacccttttattaaaggttattaccataacaccccaagcaagttatttatccctgctctctcaagccattttggaccagtttgggaagtcaatcctgcttctcacagaaagcctcattatgcaatacacatttccctaaaacttcattgttcagcatcctcattttccatatctaaaccaaactgtaaatggagttcaatacacttcctgtggagaggtgacaaattaacattaccaaaaacatgataaggctaaatttatgaaacttctagtttacctacaaaaacaaaatttccattatatatgttcatttttaagaggaaactcatgaatattagtcttgtcaaattatgtgagcatagcattcttagtgttatttttgttattctgcactatttataatttcataatttttttttttgagacggagtctcactttctcgcccaggctggagtgcagtggcaatctcggctcactgcaacctccacctcctgggttcaagtgattctcctgcctcagcctcccgagtagctgggattacaggcgcatgccaccacatccaaccaatatatatatatttggtattttttagtagagatggggtttcactgtgttggccagggtggtctcgattttctgaccccatgatccacccgccttggcctccctaagtgctgggattacaggtgtgagccaccacacccagccaatatttttcatacaattgttttttttgagacagggtctcgctctgtcacccaggctggagtgcaatggcgcgatcttggctcactgcaacctctgcctccaggctcaagtgatccacctgcctcagtctccctgaggagctgggactacaggcatgagccaccctgcctgggtaatatttctattttttttgtagagacagggttttgccatgttgtcctggctggttcaaactcctggactcaagtgacccccctgccttgggctctcaaagtgctaggattacaggcatgaaccaccacacccagcccatacactttctatatttgtattttcacttcatgtaaataaagatgcatgccatagttatttagcacacaagcatgtaaaaatataatatggtatatattcaccaacactgtggcagctttcagagtgtaagagtatgaaaactgcactttctatgggattttcattatatccatataaatattctaaggcagagtgtagagagaataattcaagtgcagagtatgattacattttcccaaaattgtatgttgattccacaaagaaaaaaaaaattgttctacatcctccaacctaaaagactgagtgtattgttattatctgctatgaagtatcctactgaggtaggataaaatgatgttggtacaaagaatgtgatttgtttatagttataagaaaacgttgaattttttttagcaaaacattatgtctgtgacacattcttaataaaactgtagcaaaatgtaattccagcaattagtgtgaattctactaaaaacaaaacaaaacaaaaaaaaccatggtattctggtttttctgaccaagctctccactctaataactgttacctcttcaatttcaaaaataagcctatttttcatcaatctctgctataaaacagctattgccattcagtagagaaagtggcaaccatttcccctgcactattcccatcacataatcagtcactaataacttattactctcctctcataaaaattccagtgtcctgaggtcttggcctgctcaatgcaggtagagccttacttccctaaaacccatggtgtctttctctcagaaaagcaccctgaacacaatcagtatgatgattgatatcatagttttacattattttctgccccaaaaccatggtctctcaattgagagaatatttaattttacaaggcagagtcctccttcttcaataaacatggataaaaatgatcctcatgtaatgaagtaagcctttccatactgtggttctttcccagataggcaccacgaaaggtgcttaaggatgcaaaatagccacagatccatagttcaggttgaaagtcacaaacagtagcctttttgagaaacctcaaacaatggaataaaagattttataacctgaaggtaagtagccatttccaaatgtcctttgacctttgaaatatataatgtcttaagttttaccatattggaacgtgtaattattgtgcagtttatcattttaaaagtgaatcaaagaactagagactgagtcactctttgtatgaatcctcacctacagttacagtcttagagtaagagcttcaggatgctcttacacattacatttgtgtggttccatcaaatacgtagattttaatgcctgcaaagctgtgaggcctgaataaagcctctgtcacacacagtacatttatgtgatttctcattattatggactcttggatgtctattaatacttgaactcatgaggagtttgccacagtcattgcattttttttttttcctttaagatggagttttgctctttttgcccaggatggagtgcattggcacgatcttggctcactgcaacctccgcctcctgggttcaagtgattctcctgcctcagcctcctatatagctgggattacaggcgcacgccaccaggcctagctaattgtgtacttttagtagaaatggggtttcgccatgttggtcaggctggtcttgaactcctgacctcaggtgatccacctgcctcggactcccaaagtgttgggattacaggcatgagccactgcacccagccagtcattgcattttcaaggaatctctcaggcataaattctctgacgttgtcaaaggaatgaattctaactgcaaaagttaccaccttcatttgtaaggtttctctccactatgaattctgtgatggcttgcaaggtttgaactctgactttagaactttccacacgttacatttgtaaggtttcccaccagtatggattgtctgatgggtagttaggcttgaacagatactaaagggtttcccacactcatatggtttctctccggtatgaattctctgatgccttgcaagttttgaagtttgactaaaggctttgccacactcattacacttgtaaggtttctctccagtatgaattccccgatgtcttgcaaggtgtgaattctgagtgaagaccttcccacactcattgcatttgtaaggtttttttccagtatggattgcctgatgggtagttaggcttgaacggacactaaaggctttcccacactgattacactcatatggtttctctccagtatgaactctctgatgccttgcaagctttgatgtttgactaaaggctttgccacattcattacactggtaaggtttacctccagtatgaactctccgatgtcttgcaaggtgtgaattctgagtgaagaccttgccacactcattacatttgtaaggtttttcaccagtatggatgacctgatgggtagttaggtttgaatgttcactaaaggctttgccatactcattatacttgtaaggtttctctccagtatgaattcgctgatgccttgaaaggtatgaattatgcctaaagaccttgccacattcattacatttataaggtttctctccagtatgaattccccgatgtcttgcaaggtgtgaattctgagtgaagaccttgccacactcattacatttgtaaggtttttctccagtatggatgacctgatgggtagttaggcttgaatacacactgaaggctttgccgcactcattacacatataaggcttcactccagtatgaattctttgatgatttgcaaggtgtgaattttgagtgaagaccttgccacattcattacatttgtaaggcttttctccagtatggatgacctgatgggtagttaggtttgaatgtgctctaaaggctttgccacactcattacacttataaggtttctctccagtatgaattagctgatgccttgcaaggtgtgaattacgcctaaagaccttgccgcattcatgacatttgtaaggcttttctccggtgtgaattaccagatgaatagctaggcttgaacgaacaccaaaggctttgccgcactcattacacttgtaaggtttctctccagtgtgaattctccagtgatttgtaaggtgtgaattttgagtgaagaccttgccacattcattacatttgtaaggtttttctccactgtgggttgcctgatggatagctaagcttgaacgagctctaaaggctttcccacactcattacacttgtaaggtttctctccagtatgaattcctcgatgtcttacaaggtgtgaattctgagtgaagaccttgccacattcgttacatttataaggtttctctccagtgtgaattttctgatgttgtgagagttgtgaatttcgactaaagaccttaccacactcattacatttgtaacgtttttcgccagtatggatcacctgatgggtagttaggtttgaacgtgttctaaaggctttgccacactcataacatttgtaaggtttctctttagtatgacttctctgatgacttgcaaggtgtgaattttgaggaaagaccatgccacatccattagatttgtaagggcttccccaattatttgctttttgcccctgtgtgagtaataaagaagagataaaatctttgagatatttcttagaaatgtgggttttgacattataaggcatttgttgaggtggtgaaactgaggaattattgttgaaagacttctcaacctgattacattcataaattttcccttcatattgaaaaagctgcagttcaggcagatgtgactgaaggcttaatccaagctgatttttaataagcttgtttcttgcatctcttttatcatgttcatctcttccatgagtgagattgccttcttgggtcaaaagcactcctttgtaatttccttcagcatctctgcattgatactcaaggccatgtgtatttttctggacttccctgaaggaacatccttcaatgtcttggctttcctgtctttccaacatcactgtttggaatacttctcctgtattactcttccctttgtgtagtaaatctttcattacaaattcggaagagagagctgtgatcacagctttgatccattcccatccatctgggtttcctgctatttgtacttggctctccaaagtgaaaggctccttcccttgctccaacatagagataatactgaggtcaaaacaagagattcccagggaggccaggttcctataattctccaacatcacgtccctgtacaaagtcctctgagcggggtccaggcatgtccactcctcctgagagaattctatagccacatccctgaatgtcacctgtccctgggtgagagccatgcctgacttgtctttctttcctcttcctcttcttcaagggttcttcgctcggcggcgtcacccgcacccaacacgatccgcttccggaact

SEQ ID NO: 15634 - RNA, 7613 nt, Homo sapiens
  source 1..7613: mol_type = other RNA
gctgggattacaggcatgagccactgtgcccagcctaatttgattattttgcttatctgtcctaagtttcctcacctctgaaatgagaatatcattaatacttatttcaggagctgatgattcagttgttacacataaagcattaataactgtgattcttactctaaatgtgattgatataaaatatatatgcaaagataaatcacttattaaagaatatatatcagttttttaaaatggaaacaaatctaaggggagtatattaaatggcagctgtcattgcaaaagttgcacaaatatcatgttttgctgtaagatcctctggctcagaaaagaaataccagccacagtaggaagttgaattgcctccagggattcaatgagagaaattatctcctttgcataaatgataattaatatcttggggactctcttattaactgtattttcatttacttctccagatgctggttaacctccacacgcttgattttcaagcatctgatctttgataacttccatattaagagacttcatttcaccatctagtatccctgtactttaattgaactaaagatttacaaggacactccattttcctatttacagagaacctagtctgtacctgccattgttttacatacattttcatgtcacaaaattttatttctaaacaacaccctcatttatgtattttctaagtgttcactggagtaacacagagaagaaatgcagtaaacatataatttggattaaaatgtatggaaggaaaaaatccttaaagtaaaaatcatatacaaaaacaaaaagtcattttactactattggctcatggctgtaatcctagcactttgggaagctgaggcaggaggaatgcttgaggccaagagttcaagaccaacctggccaacatagcgagaccccacgtctaaaaagaaaaagaaaaaaaaaaagaaaagaagctatggagaatatgttacacaataccataaactgaacaagacatgaatataacacagcctttggaaaaatgccctttggctaaaattgcttgatcatattatgtaataaacttttccacaaattcatttgcattgaactactgtaaaaatattttaggcaatttaaacagcatttcacaaatattttcaagaatgacgttgtgtaatgggccctatgggttcagcagaaaggaagagtattatctactattatgaagaaagcggaggtcttccctaacaaagaagttagaaatttcttttgtttttttgagagtctcactctattgcccaggctggagtgcagtggtgagatctcagctcactgcaacctccgtctcccgggttcaagtgattctcctgcctcagcctccctggtagctaggactacaggagtgcgccaccacacctggctaatttttgtatttttagtagagatggggtttcaccatgttggccaggctcgtcttgagctcctgacctaaggtgatccacctgcctcgggctcccaaagtgctgggattacaggcatgagcctgtaatttctggccatgcctggccagaaatcagaagttgcaagagtaaatattcagtgttgtactacagtcagtttccattttgtgatttttgtcttataccaccatttatacctctgcactccctcttcttattctgcccatctggccaagctgataatgtccgtgttccctcctttggcactagatggaagttcaaatcacgtgtgggatcctcaccccaacccacccttttattaaaggttattaccataacaccccaagcaagttatttatccctgctctctcaagccattttggaccagtttgggaagtcaatcctgcttctcacagaaagcctcattatgcaatacacatttccctaaaacttcattgttcagcatcctcattttccatatctaaaccaaactgtaaatggagttcaatacacttcctgtggagaggtgacaaattaacattaccaaaaacatgataaggctaaatttatgaaacttctagtttacctacaaaaacaaaatttccattatatatgttcatttttaagaggaaactcatgaatattagtcttgtcaaattatgtgagcatagcattcttagtgttatttttgttattctgcactatttataatttcataatttttttttttgagacggagtctcactttctcgcccaggctggagtgcagtggcaatctcggctcactgcaacctccacctcctgggttcaagtgattctcctgcctcagcctcccgagtagctgggattacaggcgcatgccaccacatccaaccaatatatatatatttggtattttttagtagagatggggtttcactgtgttggccagggtggtctcgattttctgaccccatgatccacccgccttggcctccctaagtgctgggattacaggtgtgagccaccacacccagccaatatttttcatacaattgttttttttgagacagggtctcgctctgtcacccaggctggagtgcaatggcgcgatcttggctcactgcaacctctgcctccaggctcaagtgatccacctgcctcagtctccctgaggagctgggactacaggcatgagccaccctgcctgggtaatatttctattttttttgtagagacagggttttgccatgttgtcctggctggttcaaactcctggactcaagtgacccccctgccttgggctctcaaagtgctaggattacaggcatgaaccaccacacccagcccatacactttctatatttgtattttcacttcatgtaaataaagatgcatgccatagttatttagcacacaagcatgtaaaaatataatatggtatatattcaccaacactgtggcagctttcagagtgtaagagtatgaaaactgcactttctatgggattttcattatatccatataaatattctaaggcagagtgtagagagaataattcaagtgcagagtatgattacattttcccaaaattgtatgttgattccacaaagaaaaaaaaaattgttctacatcctccaacctaaaagactgagtgtattgttattatctgctatgaagtatcctactgaggtaggataaaatgatgttggtacaaagaatgtgatttgtttatagttataagaaaacgttgaattttttttagcaaaacattatgtctgtgacacattcttaataaaactgtagcaaaatgtaattccagcaattagtgtgaattctactaaaaacaaaacaaaacaaaaaaaaccatggtattctggtttttctgaccaagctctccactctaataactgttacctcttcaatttcaaaaataagcctatttttcatcaatctctgctataaaacagctattgccattcagtagagaaagtggcaaccatttcccctgcactattcccatcacataatcagtcactaataacttattactctcctctcataaaaattccagtgtcctgaggtcttggcctgctcaatgcaggtagagccttacttccctaaaacccatggtgtctttctctcagaaaagcaccctgaacacaatcagtatgatgattgatatcatagttttacattattttctgccccaaaaccatggtctctcaattgagagaatatttaattttacaaggcagagtcctccttcttcaataaacatggataaaaatgatcctcatgtaatgaagtaagcctttccatactgtggttctttcccagataggcaccacgaaaggtgcttaaggatgcaaaatagccacagatccatagttcaggttgaaagtcacaaacagtagcctttttgagaaacctcaaacaatggaataaaagattttataacctgaaggtaagtagccatttccaaatgtcctttgacctttgaaatatataatgtcttaagttttaccatattggaacgtgtaattattgtgcagtttatcattttaaaagtgaatcaaagaactagagactgagtcactctttgtatgaatcctcacctacagttacagtcttagagtaagagcttcaggatgctcttacacattacatttgtgtggttccatcaaatacgtagattttaatgcctgcaaagctgtgaggcctgaataaagcctctgtcacacacagtacatttatgtgatttctcattattatggactcttggatgtctattaatacttgaactcatgaggagtttgccacagtcattgcattttttttttttcctttaagatggagttttgctctttttgcccaggatggagtgcattggcacgatcttggctcactgcaacctccgcctcctgggttcaagtgattctcctgcctcagcctcctatatagctgggattacaggcgcacgccaccaggcctagctaattgtgtacttttagtagaaatggggtttcgccatgttggtcaggctggtcttgaactcctgacctcaggtgatccacctgcctcggactcccaaagtgttgggattacaggcatgagccactgcacccagccagtcattgcattttcaaggaatctctcaggcataaattctctgacgttgtcaaaggaatgaattctaactgcaaaagttaccaccttcatttgtaaggtttctctccactatgaattctgtgatggcttgcaaggtttgaactctgactttagaactttccacacgttacatttgtaaggtttcccaccagtatggattgtctgatgggtagttaggcttgaacagatactaaagggtttcccacactcatatggtttctctccggtatgaattctctgatgccttgcaagttttgaagtttgactaaaggctttgccacactcattacacttgtaaggtttctctccagtatgaattccccgatgtcttgcaaggtgtgaattctgagtgaagaccttcccacactcattgcatttgtaaggtttttttccagtatggattgcctgatgggtagttaggcttgaacggacactaaaggctttcccacactgattacactcatatggtttctctccagtatgaactctctgatgccttgcaagctttgatgtttgactaaaggctttgccacattcattacactggtaaggtttacctccagtatgaactctccgatgtcttgcaaggtgtgaattctgagtgaagaccttgccacactcattacatttgtaaggtttttcaccagtatggatgacctgatgggtagttaggtttgaatgttcactaaaggctttgccatactcattatacttgtaaggtttctctccagtatgaattcgctgatgccttgaaaggtatgaattatgcctaaagaccttgccacattcattacatttataaggtttctctccagtatgaattccccgatgtcttgcaaggtgtgaattctgagtgaagaccttgccacactcattacatttgtaaggtttttctccagtatggatgacctgatgggtagttaggcttgaatacacactgaaggctttgccgcactcattacacatataaggcttcactccagtatgaattctttgatgatttgcaaggtgtgaattttgagtgaagaccttgccacattcattacatttgtaaggcttttctccagtatggatgacctgatgggtagttaggtttgaatgtgctctaaaggctttgccacactcattacacttataaggtttctctccagtatgaattagctgatgccttgcaaggtgtgaattacgcctaaagaccttgccgcattcatgacatttgtaaggcttttctccggtgtgaattaccagatgaatagctaggcttgaacgaacaccaaaggctttgccgcactcattacacttgtaaggtttctctccagtgtgaattctccagtgatttgtaaggtgtgaattttgagtgaagaccttgccacattcattacatttgtaaggtttttctccactgtgggttgcctgatggatagctaagcttgaacgagctctaaaggctttcccacactcattacacttgtaaggtttctctccagtatgaattcctcgatgtcttacaaggtgtgaattctgagtgaagaccttgccacattcgttacatttataaggtttctctccagtgtgaattttctgatgttgtgagagttgtgaatttcgactaaagaccttaccacactcattacatttgtaacgtttttcgccagtatggatcacctgatgggtagttaggtttgaacgtgttctaaaggctttgccacactcataacatttgtaaggtttctctttagtatgacttctctgatgacttgcaaggtgtgaattttgaggaaagaccatgccacatccattagatttgtaagggcttccccaattatttgctttttgcccctgtgtgagtaataaagaagagataaaatctttgagatatttcttagaaatgtgggttttgacattataaggcatttgttgaggtggtgaaactgaggaattattgttgaaagacttctcaacctgattacattcataaattttcccttcatattgaaaaagctgcagttcaggcagatgtgactgaaggcttaatccaagctgatttttaataagcttgtttcttgcatctcttttatcatgttcatctcttccatgagtgagattgccttcttgggtcaaaagcactcctttgtaatttccttcagcatctctgcattgatactcaaggccatgtgtatttttctggacttccctgaaggaacatccttcaatgtcttggctttcctgtctttccaacatcactgtttggaatacttctcctgtattactcttccctttgtgtagtaaatctttcattacaaattcggaagagagagctgtgatcacagctttgatccattcccatccatctgggtttcctgctatttgtacttggctctccaaagtgaaaggctccttcccttgctccaacatagagataatactgaggtcaaaacaagagattcctgccagggaggccaggttcctataattctccaacatcacgtccctgtacaaagtcctctgagcggggtccaggcatgtccactcctcctgagagaattctatagccacatccctgaatgtcacctgtccctgggtgagagccatgcctgacttgtctttctttcctcttcctcttcttcaagggttcttcctgaggtcaggagttcgagatcagcctgggcaacacggtgaaaccccgtctctactaaaaatacaaaattagccgggcgtggtggcacatgcctgtaatcccagctactcgggaggctgaggcaggagaatcgcttgaacctgggaggcggaggatgcggtgagccgaaatcgcgccattgcactccagcctggacaacaagagtaaatctccgtctcaccaaaaaaaaaaaaaaagaaaaaaaaaaaggtctgtagcgagcccgggaactggctgcggaaacggggcacggcggttcgcaagtttaatccatactgagggacactcacgctcggcggcgtcacccgcacccaacacgatccgcttccggaact

SEQ ID NO: 15635 - RNA, 7284 nt, Homo sapiens
  source 1..7284: mol_type = other RNA
gctgggattacaggcatgagccactgtgcccagcctaatttgattattttgcttatctgtcctaagtttcctcacctctgaaatgagaatatcattaatacttatttcaggagctgatgattcagttgttacacataaagcattaataactgtgattcttactctaaatgtgattgatataaaatatatatgcaaagataaatcacttattaaagaatatatatcagttttttaaaatggaaacaaatctaaggggagtatattaaatggcagctgtcattgcaaaagttgcacaaatatcatgttttgctgtaagatcctctggctcagaaaagaaataccagccacagtaggaagttgaattgcctccagggattcaatgagagaaattatctcctttgcataaatgataattaatatcttggggactctcttattaactgtattttcatttacttctccagatgctggttaacctccacacgcttgattttcaagcatctgatctttgataacttccatattaagagacttcatttcaccatctagtatccctgtactttaattgaactaaagatttacaaggacactccattttcctatttacagagaacctagtctgtacctgccattgttttacatacattttcatgtcacaaaattttatttctaaacaacaccctcatttatgtattttctaagtgttcactggagtaacacagagaagaaatgcagtaaacatataatttggattaaaatgtatggaaggaaaaaatccttaaagtaaaaatcatatacaaaaacaaaaagtcattttactactattggctcatggctgtaatcctagcactttgggaagctgaggcaggaggaatgcttgaggccaagagttcaagaccaacctggccaacatagcgagaccccacgtctaaaaagaaaaagaaaaaaaaaaagaaaagaagctatggagaatatgttacacaataccataaactgaacaagacatgaatataacacagcctttggaaaaatgccctttggctaaaattgcttgatcatattatgtaataaacttttccacaaattcatttgcattgaactactgtaaaaatattttaggcaatttaaacagcatttcacaaatattttcaagaatgacgttgtgtaatgggccctatgggttcagcagaaaggaagagtattatctactattatgaagaaagcggaggtcttccctaacaaagaagttagaaatttcttttgtttttttgagagtctcactctattgcccaggctggagtgcagtggtgagatctcagctcactgcaacctccgtctcccgggttcaagtgattctcctgcctcagcctccctggtagctaggactacaggagtgcgccaccacacctggctaatttttgtatttttagtagagatggggtttcaccatgttggccaggctcgtcttgagctcctgacctaaggtgatccacctgcctcgggctcccaaagtgctgggattacaggcatgagcctgtaatttctggccatgcctggccagaaatcagaagttgcaagagtaaatattcagtgttgtactacagtcagtttccattttgtgatttttgtcttataccaccatttatacctctgcactccctcttcttattctgcccatctggccaagctgataatgtccgtgttccctcctttggcactagatggaagttcaaatcacgtgtgggatcctcaccccaacccacccttttattaaaggttattaccataacaccccaagcaagttatttatccctgctctctcaagccattttggaccagtttgggaagtcaatcctgcttctcacagaaagcctcattatgcaatacacatttccctaaaacttcattgttcagcatcctcattttccatatctaaaccaaactgtaaatggagttcaatacacttcctgtggagaggtgacaaattaacattaccaaaaacatgataaggctaaatttatgaaacttctagtttacctacaaaaacaaaatttccattatatatgttcatttttaagaggaaactcatgaatattagtcttgtcaaattatgtgagcatagcattcttagtgttatttttgttattctgcactatttataatttcataatttttttttttgagacggagtctcactttctcgcccaggctggagtgcagtggcaatctcggctcactgcaacctccacctcctgggttcaagtgattctcctgcctcagcctcccgagtagctgggattacaggcgcatgccaccacatccaaccaatatatatatatttggtattttttagtagagatggggtttcactgtgttggccagggtggtctcgattttctgaccccatgatccacccgccttggcctccctaagtgctgggattacaggtgtgagccaccacacccagccaatatttttcatacaattgttttttttgagacagggtctcgctctgtcacccaggctggagtgcaatggcgcgatcttggctcactgcaacctctgcctccaggctcaagtgatccacctgcctcagtctccctgaggagctgggactacaggcatgagccaccctgcctgggtaatatttctattttttttgtagagacagggttttgccatgttgtcctggctggttcaaactcctggactcaagtgacccccctgccttgggctctcaaagtgctaggattacaggcatgaaccaccacacccagcccatacactttctatatttgtattttcacttcatgtaaataaagatgcatgccatagttatttagcacacaagcatgtaaaaatataatatggtatatattcaccaacactgtggcagctttcagagtgtaagagtatgaaaactgcactttctatgggattttcattatatccatataaatattctaaggcagagtgtagagagaataattcaagtgcagagtatgattacattttcccaaaattgtatgttgattccacaaagaaaaaaaaaattgttctacatcctccaacctaaaagactgagtgtattgttattatctgctatgaagtatcctactgaggtaggataaaatgatgttggtacaaagaatgtgatttgtttatagttataagaaaacgttgaattttttttagcaaaacattatgtctgtgacacattcttaataaaactgtagcaaaatgtaattccagcaattagtgtgaattctactaaaaacaaaacaaaacaaaaaaaaccatggtattctggtttttctgaccaagctctccactctaataactgttacctcttcaatttcaaaaataagcctatttttcatcaatctctgctataaaacagctattgccattcagtagagaaagtggcaaccatttcccctgcactattcccatcacataatcagtcactaataacttattactctcctctcataaaaattccagtgtcctgaggtcttggcctgctcaatgcaggtagagccttacttccctaaaacccatggtgtctttctctcagaaaagcaccctgaacacaatcagtatgatgattgatatcatagttttacattattttctgccccaaaaccatggtctctcaattgagagaatatttaattttacaaggcagagtcctccttcttcaataaacatggataaaaatgatcctcatgtaatgaagtaagcctttccatactgtggttctttcccagataggcaccacgaaaggtgcttaaggatgcaaaatagccacagatccatagttcaggttgaaagtcacaaacagtagcctttttgagaaacctcaaacaatggaataaaagattttataacctgaaggtaagtagccatttccaaatgtcctttgacctttgaaatatataatgtcttaagttttaccatattggaacgtgtaattattgtgcagtttatcattttaaaagtgaatcaaagaactagagactgagtcactctttgtatgaatcctcacctacagttacagtcttagagtaagagcttcaggatgctcttacacattacatttgtgtggttccatcaaatacgtagattttaatgcctgcaaagctgtgaggcctgaataaagcctctgtcacacacagtacatttatgtgatttctcattattatggactcttggatgtctattaatacttgaactcatgaggagtttgccacagtcattgcattttttttttttcctttaagatggagttttgctctttttgcccaggatggagtgcattggcacgatcttggctcactgcaacctccgcctcctgggttcaagtgattctcctgcctcagcctcctatatagctgggattacaggcgcacgccaccaggcctagctaattgtgtacttttagtagaaatggggtttcgccatgttggtcaggctggtcttgaactcctgacctcaggtgatccacctgcctcggactcccaaagtgttgggattacaggcatgagccactgcacccagccagtcattgcattttcaaggaatctctcaggcataaattctctgacgttgtcaaaggaatgaattctaactgcaaaagttaccaccttcatttgtaaggtttctctccactatgaattctgtgatggcttgcaaggtttgaactctgactttagaactttccacacgttacatttgtaaggtttcccaccagtatggattgtctgatgggtagttaggcttgaacagatactaaagggtttcccacactcatatggtttctctccggtatgaattctctgatgccttgcaagttttgaagtttgactaaaggctttgccacactcattacacttgtaaggtttctctccagtatgaattccccgatgtcttgcaaggtgtgaattctgagtgaagaccttcccacactcattgcatttgtaaggtttttttccagtatggattgcctgatgggtagttaggcttgaacggacactaaaggctttcccacactgattacactcatatggtttctctccagtatgaactctctgatgccttgcaagctttgatgtttgactaaaggctttgccacattcattacactggtaaggtttacctccagtatgaactctccgatgtcttgcaaggtgtgaattctgagtgaagaccttgccacactcattacatttgtaaggtttttcaccagtatggatgacctgatgggtagttaggtttgaatgttcactaaaggctttgccatactcattatacttgtaaggtttctctccagtatgaattcgctgatgccttgaaaggtatgaattatgcctaaagaccttgccacattcattacatttataaggtttctctccagtatgaattccccgatgtcttgcaaggtgtgaattctgagtgaagaccttgccacactcattacatttgtaaggtttttctccagtatggatgacctgatgggtagttaggcttgaatacacactgaaggctttgccgcactcattacacatataaggcttcactccagtatgaattctttgatgatttgcaaggtgtgaattttgagtgaagaccttgccacattcattacatttgtaaggcttttctccagtatggatgacctgatgggtagttaggtttgaatgtgctctaaaggctttgccacactcattacacttataaggtttctctccagtatgaattagctgatgccttgcaaggtgtgaattacgcctaaagaccttgccgcattcatgacatttgtaaggcttttctccggtgtgaattaccagatgaatagctaggcttgaacgaacaccaaaggctttgccgcactcattacacttgtaaggtttctctccagtgtgaattctccagtgatttgtaaggtgtgaattttgagtgaagaccttgccacattcattacatttgtaaggtttttctccactgtgggttgcctgatggatagctaagcttgaacgagctctaaaggctttcccacactcattacacttgtaaggtttctctccagtatgaattcctcgatgtcttacaaggtgtgaattctgagtgaagaccttgccacattcgttacatttataaggtttctctccagtgtgaattttctgatgttgtgagagttgtgaatttcgactaaagaccttaccacactcattacatttgtaacgtttttcgccagtatggatcacctgatgggtagttaggtttgaacgtgttctaaaggctttgccacactcataacatttgtaaggtttctctttagtatgacttctctgatgacttgcaaggtgtgaattttgaggaaagaccatgccacatccattagatttgtaagggcttccccaattatttgctttttgcccctgtgtgagtaataaagaagagataaaatctttgagatatttcttagaaatgtgggttttgacattataaggcatttgttgaggtggtgaaactgaggaattattgttgaaagacttctcaacctgattacattcataaattttcccttcatattgaaaaagctgcagttcaggcagatgtgactgaaggcttaatccaagctgatttttaataagcttgtttcttgcatctcttttatcatgttcatctcttccatgagtgagattgccttcttgggtcaaaagcactcctttgtaatttccttcagcatctctgcattgatactcaaggccatgtgtatttttctggacttccctgaaggaacatccttcaatgtcttggctttcctgtctttccaacatcactgtttggaatacttctcctgtattactcttccctttgtgtagtaaatctttcattacaaattcggaagagagagctgtgatcacagctttgatccattcccatccatctgggtttcctgctatttgtacttggctctccaaagtgaaaggctccttcccttgctccaacatagagataatactgaggtcaaaacaagagattcctgccagggaggccaggttcctataattctccaacatcacgtccctgtacaaagtcctctgagcggggtccaggcatgtccactcctcctgagagaattctatagccacatccctgaatgtcacctgtccctgggtgagagccatgcctgacttgtctttctttcctcttcctcttcttcaagggttcttcgctcggcggcgtcacccgcacccaacacgatccgcttccggaact

SEQ ID NO: 15636 - RNA, 3341 nt, Homo sapiens
  source 1..3341: mol_type = other RNA
gctgggattacaggcatgagccactgtgcccagcctagactctttaagtggtaacagaaacccaaatcaaacaagcttaagcaaaataaggaaattacttttgtctcaaaaccagaaagcttaataatgtgtggttggatctggaggttcgaataatagtacttactttgtccactgctgggtctcattttcagagaaactttacatttgataatattgcagttgttacagttggtagccttgaacccacatcattccttcatctggcatgccccttctcccaccccctgcaaaaagaaagtctagtctggcagaagtctgattggcccaaggaatgctgtgtgctcagcattaaggttggtggtcttgtgcagggaaaggatggatccctactcttacctacttcatggaatgaacaggatttttgtggaatggaggaggcatgtttcccctgatgaaggaatttttgacatacaaaaaatattctttttttattaaaaattttaatcaaaaaataatatggaataaaaataatagggaataaacattaaaagttggttacttgttcagcactccttattcccaggaacgaggcatttctctaataagatatgatggggttgcactgtgaagttcattgattattaaagggtgaacgatttatcagctacagtaggtaagatggatatgacatctacattttagaattcatagaaagacttagagacccaaatatgtattttccatactaaatgctacatttttgagatacatatccatatataagtgattatattctatctacctcatctaagacaaaataaaaattagaactcagcagccagagtagaatagtaaaaacactgactttggagtcagaagttgggttggagtgtttgccaattgctaattacaacttttgtcaaataattaacttttcttaacatcttccagaagtgaaatagagctgatcctatcttacaagattattgtgaagattaaatgacatcgtgtatttttgagagaagagaataagtaacatgatgaagcatgtcattagagggagatcattatctatttagcattaatttctgtatcaacacccaaaacttttttttaaaacaacagaagcttgtcagtatggaatcttaaaaactacacgtgttatcttacctcataatctactgtctttgactgaagtgggactcttctttacagatccatacggaggtattccatagagatgctttgctgcttttgtggacaagcagcctgtggcagatgcagttttacacacatagttttgcttcaccagccatttccatgaagggtaacagatacaaatcaggaacccagactgtgttcattgtatgattcagggaggtttccacacagaactcacgctgttttcagatgggtaagcgagtgtgtcaatgagagtagtccacgaatgcagaatgatccttttctgatttcactgatcaaataagttaaccccatgtaaacatcagactgtcttgttctccctaggcttgcttttcattctttggtatgacagttctgattcttcagcctccccatgaagaaaagaaaaattctcttgaagctgaactaaattcatcagcaaatgaaattatattcatttgataaaatgctaaatggaaaaggcaggtttattttaagccgtcaacaggctgttttagttaatcatgcacagtgcagaagacaggagtttggttgctaagaaaatgtttggcatgtttccacgagatccatgtgacgtgaaatgcatctgttcatttcaatagtgaaatagaaaaaaataaaataaacagtgcagggtatatttggtgagtcactgtggaacacagggccaaaataacttctgtgttgtcagtttattctatacaaccttattgttatgatgttagccttttcttataattcaaaaaaaatttattttaatagtgatgttttgttagcaaattaatacaaattcattgtagataaatcagaaaatacaaaataagaaaattaaaatctgctgtaacacacacccacacaaataccaatatctatattggtatgtgcatagtaggggcttaatatttatttgctaaatgaattaatatatattttacttacaaatatgagatcatactgtaatacttttataacatgctttagaaattaaaagacatcataaacatttttactgtgttattaagtattcttctttagcataattgtaatagttttcattattatgggacaagtaagttatctggaactcctgcaaaatttcttcagtagccaggaactgaatgcgagcacctcccagtaagactgatactgtggtgctgatatgatgaaatctgaacatgttcaacattttttgctgggatgtcatacatattctctgattactgagctagtaaatggaatctcagctgtcctgattgtgtgtaattctgtcatttctaccaccagatagagaccatcactgcttacatagataacgtgccattcacatccaggtgtactaatgtgagagagaatggccaaagatagcaatgtgcttggcacacccttgcacgccatcgtgatcctcagagtgaagtaagaatggctattgtcttccacaacatcttcaaggttgctgcaggggaagagctcctctgtcacaaggtgcctcatctgaagccactattaaagcgggtgtccatgctgaccagaaacaaagcacatttcacagacctattaacagttggaggcaggtgtttcctggttggtggacgtttcttctccacttagcaactcagggacacaaactgattttgccttctctttgtcagggcttcaaattcatcatctgcctccagtcagtgaaagaaaaatgagagcttggaggtggaacacctccttctttaaagctctgtcccagaaattgtattcattactagaactcagtcatgtgatctaactgcaagaaggctgggatatgtagtccaattgtgtacccaagaacagaaaatggtttgttagggaggggagaaacagcaaccattatctgaggttgcttaaatttggtcatattttgaatactttagtacatgctggcagtgctgtaaataagcaaaaatgaatccggcacccacattctgattgccaccaacttcgtgtaattttttaaaggtatataaaattcatgtgtcaatgcataaagatccattttaaattgataccataaaaaacaagtggaattgctgggtcaaatattcatacagaattctctggcttttcattaagtcgtgtctaattgaccctgagaaattgttcaa

SEQ ID NO: 15637 - RNA, 3209 nt, Homo sapiens
  source 1..3209: mol_type = other RNA
gctgggattacaggcatgagccactgtgcccagcctagactctttaagtggtaacagaaacccaaatcaaacaagcttaagcaaaataaggaaattacttttgtctcaaaaccagaaagcttaataatgtgtggttggatctggaggttcgaataatagtacttactttgtccactgctgggtctcattttcagagaaactttacatttgataatattgcagttgttacagttggtagccttgaacccacatcattccttcatctggcatgccccttctcccaccccctgcaaaaagaaagtctagtctggcagaagtctgattggcccaaggaatgctgtgtgctcagcattaaggttggtggtcttgtgcagggaaaggatggatccctactcttacctacttcatggaatgaacaggatttttgtggaatggaggaggcatgtttcccctgatgaaggaatttttgacatacaaaaaatattctttttttattaaaaattttaatcaaaaaataatatggaataaaaataatagggaataaacattaaaagttggttacttgttcagcactccttattcccaggaacgaggcatttctctaataagatatgatggggttgcactgtgaagttcattgattattaaagggtgaacgatttatcagctacagtaggtaagatggatatgacatctacattttagaattcatagaaagacttagagacccaaatatgtattttccatactaaatgctacatttttgagatacatatccatatataagtgattatattctatctacctcatctaagacaaaataaaaattagaactcagcagccagagtagaatagtaaaaacactgactttggagtcagaagttgggttggagtgtttgccaattgctaattacaacttttgtcaaataattaacttttcttaacatcttccagaagtgaaatagagctgatcctatcttacaagattattgtgaagattaaatgacatcgtgtatttttgagagaagagaataagtaacatgatgaagcatgtcattagagggagatcattatctatttagcattaatttctgtatcaacacccaaaacttttttttaaaacaacagaagcttgtcagtatggaatcttaaaaactacacgtgttatcttacctcataatctactgtctttgactgaagtgggactcttctttacagatccatacggaggtattccatagagatgctttgctgcttttgtggacaagcagcctgtggcagatgcagttttacacacatagttttgcttcaccagccatttccatgaagggtaacagatacaaatcaggaacccagactgtgttccatgtaaacatcagactgtcttgttctccctaggcttgcttttcattctttggtatgacagttctgattcttcagcctccccatgaagaaaagaaaaattctcttgaagctgaactaaattcatcagcaaatgaaattatattcatttgataaaatgctaaatggaaaaggcaggtttattttaagccgtcaacaggctgttttagttaatcatgcacagtgcagaagacaggagtttggttgctaagaaaatgtttggcatgtttccacgagatccatgtgacgtgaaatgcatctgttcatttcaatagtgaaatagaaaaaaataaaataaacagtgcagggtatatttggtgagtcactgtggaacacagggccaaaataacttctgtgttgtcagtttattctatacaaccttattgttatgatgttagccttttcttataattcaaaaaaaatttattttaatagtgatgttttgttagcaaattaatacaaattcattgtagataaatcagaaaatacaaaataagaaaattaaaatctgctgtaacacacacccacacaaataccaatatctatattggtatgtgcatagtaggggcttaatatttatttgctaaatgaattaatatatattttacttacaaatatgagatcatactgtaatacttttataacatgctttagaaattaaaagacatcataaacatttttactgtgttattaagtattcttctttagcataattgtaatagttttcattattatgggacaagtaagttatctggaactcctgcaaaatttcttcagtagccaggaactgaatgcgagcacctcccagtaagactgatactgtggtgctgatatgatgaaatctgaacatgttcaacattttttgctgggatgtcatacatattctctgattactgagctagtaaatggaatctcagctgtcctgattgtgtgtaattctgtcatttctaccaccagatagagaccatcactgcttacatagataacgtgccattcacatccaggtgtactaatgtgagagagaatggccaaagatagcaatgtgcttggcacacccttgcacgccatcgtgatcctcagagtgaagtaagaatggctattgtcttccacaacatcttcaaggttgctgcaggggaagagctcctctgtcacaaggtgcctcatctgaagccactattaaagcgggtgtccatgctgaccagaaacaaagcacatttcacagacctattaacagttggaggcaggtgtttcctggttggtggacgtttcttctccacttagcaactcagggacacaaactgattttgccttctctttgtcagggcttcaaattcatcatctgcctccagtcagtgaaagaaaaatgagagcttggaggtggaacacctccttctttaaagctctgtcccagaaattgtattcattactagaactcagtcatgtgatctaactgcaagaaggctgggatatgtagtccaattgtgtacccaagaacagaaaatggtttgttagggaggggagaaacagcaaccattatctgaggttgcttaaatttggtcatattttgaatactttagtacatgctggcagtgctgtaaataagcaaaaatgaatccggcacccacattctgattgccaccaacttcgtgtaattttttaaaggtatataaaattcatgtgtcaatgcataaagatccattttaaattgataccataaaaaacaagtggaattgctgggtcaaatattcatacagaattctctggcttttcattaagtcgtgtctaattgaccctgagaaattgttcaa

SEQ ID NO: 15638 - RNA, 3300 nt, Homo sapiens
  source 1..3300: mol_type = other RNA
gctgggattacaggcatgagccactgtgcccagcctagactctttaagtggtaacagaaacccaaatcaaacaagcttaagcaaaataaggaaattacttttgtctcaaaaccagaaagcttaataatgtgtggttggatctggaggttcgaataatagtacttactttgtccactgctgggtctcattttcagagaaactttacatttgataatattgcagttgttacagttggtagccttgaacccacatcattccttcatctggcatgccccttctcccaccccctgcaaaaagaaagtctagtctggcagaagtctgattggcccaaggaatgctgtgtgctcagcattaaggttggtggtcttgtgcagggaaaggatggatccctactcttacctacttcatggaatgaacaggatttttgtggaatggaggaggcatgtttcccctgatgaaggaatttttgacatacaaaaaatattctttttttattaaaaattttaatcaaaaaataatatggaataaaaataatagggaataaacattaaaagttggttacttgttcagcactccttattcccaggaacgaggcatttctctaataagatatgatggggttgcactgtgaagttcattgattattaaagggtgaacgatttatcagctacagtaggtaagatggatatgacatctacattttagaattcatagaaagacttagagacccaaatatgtattttccatactaaatgctacatttttgagatacatatccatatataagtgattatattctatctacctcatctaagacaaaataaaaattagaactcagcagccagagtagaatagtaaaaacactgactttggagtcagaagttgggttggagtgtttgccaattgctaattacaacttttgtcaaataattaacttttcttaacatcttccagaagtgaaatagagctgatcctatcttacaagattattgtgaagattaaatgacatcgtgtatttttgagagaagagaataagtaacatgatgaagcatgtcattagagggagatcattatctatttagcattaatttctgtatcaacacccaaaacttttttttaaaacaacagaagcttgtcagtatggaatcttaaaaactacacgtgttatcttacctcataatctactgtctttgactgaagtgggactcttctttacagatccatacggaggtattccatagagatgctttgctgcttttgtggacaagcagcctgtggcagatgcagttttacacacatagttttgcttcaccagccatttccatgaagggtaacagatacaaatcaggaacccagactgtgttgctgttttcagatgggtaagcgagtgtgtcaatgagagtagtccacgaatgcagaatgatccttttctgatttcactgatcaaataagttaaccccatgtaaacatcagactgtcttgttctccctaggcttgcttttcattctttggtatgacagttctgattcttcagcctccccatgaagaaaagaaaaattctcttgaagctgaactaaattcatcagcaaatgaaattatattcatttgataaaatgctaaatggaaaaggcaggtttattttaagccgtcaacaggctgttttagttaatcatgcacagtgcagaagacaggagtttggttgctaagaaaatgtttggcatgtttccacgagatccatgtgacgtgaaatgcatctgttcatttcaatagtgaaatagaaaaaaataaaataaacagtgcagggtatatttggtgagtcactgtggaacacagggccaaaataacttctgtgttgtcagtttattctatacaaccttattgttatgatgttagccttttcttataattcaaaaaaaatttattttaatagtgatgttttgttagcaaattaatacaaattcattgtagataaatcagaaaatacaaaataagaaaattaaaatctgctgtaacacacacccacacaaataccaatatctatattggtatgtgcatagtaggggcttaatatttatttgctaaatgaattaatatatattttacttacaaatatgagatcatactgtaatacttttataacatgctttagaaattaaaagacatcataaacatttttactgtgttattaagtattcttctttagcataattgtaatagttttcattattatgggacaagtaagttatctggaactcctgcaaaatttcttcagtagccaggaactgaatgcgagcacctcccagtaagactgatactgtggtgctgatatgatgaaatctgaacatgttcaacattttttgctgggatgtcatacatattctctgattactgagctagtaaatggaatctcagctgtcctgattgtgtgtaattctgtcatttctaccaccagatagagaccatcactgcttacatagataacgtgccattcacatccaggtgtactaatgtgagagagaatggccaaagatagcaatgtgcttggcacacccttgcacgccatcgtgatcctcagagtgaagtaagaatggctattgtcttccacaacatcttcaaggttgcaggggaagagctcctctgtcacaaggtgcctcatctgaagccactattaaagcgggtgtccatgctgaccagaaacaaagcacatttcacagacctattaacagttggaggcaggtgtttcctggttggtggacgtttcttctccacttagcaactcagggacacaaactgattttgccttctctttgtcagggcttcaaattcatcatctgcctccagtcagtgaaagaaaaatgagagcttggaggtggaacacctccttctttaaagctctgtcccagaaattgtattcattactagaactcagtcatgtgatctaactgcaagaaggctgggatatgtagtccaattgtgtacccaagaacagaaaatggtttgttagggaggggagaaacagcaaccattatctgaggttgcttaaatttggtcatattttgaatactttagtacatgctggcagtgctgtaaataagcaaaaatgaatccggcacccacattctgattgccaccaacttcgtgtaattttttaaaggtatataaaattcatgtgtcaatgcataaagatccattttaaattgataccataaaaaacaagtggaattgctgggtcaaatattcatacagaattctctggcttttcattaagtcgtgtctaattgaccctgagaaattgttcaa

SEQ ID NO: 15639 - RNA, 3283 nt, Homo sapiens
  source 1..3283: mol_type = other RNA
gctgggattacaggcatgagccactgtgcccagcctagactctttaagtggtaacagaaacccaaatcaaacaagcttaagcaaaataaggaaattacttttgtctcaaaaccagaaagcttaataatgtgtggttggatctggaggttcgaataatagtacttactttgtccactgctgggtctcattttcagagaaactttacatttgataatattgcagttgttacagttggtagccttgaacccacatcattccttcatctggcatgccccttctcccaccccctgcaaaaagaaagtctagtctggcagaagtctgattggcccaaggaatgctgtgtgctcagcattaaggttggtggtcttgtgcagggaaaggatggatccctactcttacctacttcatggaatgaacaggatttttgtggaatggaggaggcatgtttcccctgatgaaggaatttttgacatacaaaaaatattctttttttattaaaaattttaatcaaaaaataatatggaataaaaataatagggaataaacattaaaagttggttacttgttcagcactccttattcccaggaacgaggcatttctctaataagatatgatggggttgcactgtgaagttcattgattattaaagggtgaacgatttatcagctacagtaggtaagatggatatgacatctacattttagaattcatagaaagacttagagacccaaatatgtattttccatactaaatgctacatttttgagatacatatccatatataagtgattatattctatctacctcatctaagacaaaataaaaattagaactcagcagccagagtagaatagtaaaaacactgactttggagtcagaagttgggttggagtgtttgccaattgctaattacaacttttgtcaaataattaacttttcttaacatcttccagaagtgaaatagagctgatcctatcttacaagattattgtgaagattaaatgacatcgtgtatttttgagagaagagaataagtaacatgatgaagcatgtcattagagggagatcattatctatttagcattaatttctgtatcaacacccaaaacttttttttaaaacaacagaagcttgtcagtatggaatcttaaaaactacacgtgttatcttacctcataatctactgtctttgactgaagtgggactcttctttacagatccatacggaggtattccatagagatgctttgctgcttttgtggacaagcagcctgtggcagatgcagttttacacacatagttttgcttcaccagccatttccatgaagggtaacagatacaaatcaggaacccagactgtgttgctgttttcagatgggtaagcgagtgtgtcaatgagagtagtccacgaatgcagaatgatccttttctgatttcactgatcaaataagttaaccccatgtaaacatcagactgtcttgttctccctaggcttgcttttcattctttggtatgacagttctgattcttcagcctccccatgaagaaaagaaaaattctcttgaagctgaactaaattcatcagcaaatgaaattatattcatttgataaaatgctaaatggaaaaggcaggtttattttaagccgtcaacaggctgttttagttaatcatgcacagtgcagaagacaggagtttggttgctaagaaaatgtttggcatgtttccacgagatccatgtgacgtgaaatgcatctgttcatttcaatagtgaaatagaaaaaaataaaataaacagtgcagggtatatttggtgagtcactgtggaacacagggccaaaataacttctgtgttgtcagtttattctatacaaccttattgttatgatgttagccttttcttataattcaaaaaaaatttattttaatagtgatgttttgttagcaaattaatacaaattcattgtagataaatcagaaaatacaaaataagaaaattaaaatctgctgtaacacacacccacacaaataccaatatctatattggtatgtgcatagtaggggcttaatatttatttgctaaatgaattaatatatattttacttacaaatatgagatcatactgtaatacttttataacatgctttagaaattaaaagacatcataaacatttttactgtgttattaagtattcttctttagcataattgtaatagttttcattattatgggacaagtaagttatctggaactcctgcaaaatttcttcagtagccaggaactgaatgcgagcacctcccagtaagactgatactgtggtgctgatatgatgaaatctgaacatgttcaacattttttgctgggatgtcatacatattctctgattactgagctagtaaatggaatctcagctgtcctgattgtgtgtaattctgtcatttctaccaccagatagagaccatcactgcttacatagataacgtgccattcacatccaggtgtactaatgtgagagagaatggccaaagatagcaatgtgcttggcacacccttgcacgccatcgtgatcctcagagtgaagtaagaatggctattgtcttccacaacatcttcaaggttgctgcaggggaagagctcctctgtcacaaggtgcctcatctgaagccactattaaagcgggtgtccatgctgaccagaaacaaagcacatttcacagacctactgcagtaggtgagagtagctgccttctgtgctatcatcgacatcattgttaacattgcatacagcattcacattttaaagttttttaagagacacattatgatatggtaattgagagaacagaccctaaatccatactgcctggatccgaattccaccttgtcttttttcttcctgagacctttctgtgtctcagttttcttatcaaggattcagtgacaattcgtgtggacaatttatgtcatcaaattcagaatgccaccatggcagatatcaccaatgccgattcaaaacccatatttaggcaccaggaactttctcaggtccactctgacacagaaattgcatacaacatgtcaggttctctggacaatggtactgatgtctgagcataggcatgtccttggctgtgcctgccagtgatgcagggtattttctcaaccccttcataggacttgtggcaagggtgcctcatttactcagcctgctctgctcaacccctctcgggagggagtgtgcaagcaagcgagtgtggaatcagagttagcaagtgcaagagct

SEQ ID NO: 15640 - RNA, 3303 nt, Homo sapiens
  source 1..3303: mol_type = other RNA
gctgggattacaggcatgagccactgtgcccagcctagactctttaagtggtaacagaaacccaaatcaaacaagcttaagcaaaataaggaaattacttttgtctcaaaaccagaaagcttaataatgtgtggttggatctggaggttcgaataatagtacttactttgtccactgctgggtctcattttcagagaaactttacatttgataatattgcagttgttacagttggtagccttgaacccacatcattccttcatctggcatgccccttctcccaccccctgcaaaaagaaagtctagtctggcagaagtctgattggcccaaggaatgctgtgtgctcagcattaaggttggtggtcttgtgcagggaaaggatggatccctactcttacctacttcatggaatgaacaggatttttgtggaatggaggaggcatgtttcccctgatgaaggaatttttgacatacaaaaaatattctttttttattaaaaattttaatcaaaaaataatatggaataaaaataatagggaataaacattaaaagttggttacttgttcagcactccttattcccaggaacgaggcatttctctaataagatatgatggggttgcactgtgaagttcattgattattaaagggtgaacgatttatcagctacagtaggtaagatggatatgacatctacattttagaattcatagaaagacttagagacccaaatatgtattttccatactaaatgctacatttttgagatacatatccatatataagtgattatattctatctacctcatctaagacaaaataaaaattagaactcagcagccagagtagaatagtaaaaacactgactttggagtcagaagttgggttggagtgtttgccaattgctaattacaacttttgtcaaataattaacttttcttaacatcttccagaagtgaaatagagctgatcctatcttacaagattattgtgaagattaaatgacatcgtgtatttttgagagaagagaataagtaacatgatgaagcatgtcattagagggagatcattatctatttagcattaatttctgtatcaacacccaaaacttttttttaaaacaacagaagcttgtcagtatggaatcttaaaaactacacgtgttatcttacctcataatctactgtctttgactgaagtgggactcttctttacagatccatacggaggtattccatagagatgctttgctgcttttgtggacaagcagcctgtggcagatgcagttttacacacatagttttgcttcaccagccatttccatgaagggtaacagatacaaatcaggaacccagactgtgttgctgttttcagatgggtaagcgagtgtgtcaatgagagtagtccacgaatgcagaatgatccttttctgatttcactgatcaaataagttaaccccatgtaaacatcagactgtcttgttctccctaggcttgcttttcattctttggtatgacagttctgattcttcagcctccccatgaagaaaagaaaaattctcttgaagctgaactaaattcatcagcaaatgaaattatattcatttgataaaatgctaaatggaaaaggcaggtttattttaagccgtcaacaggctgttttagttaatcatgcacagtgcagaagacaggagtttggttgctaagaaaatgtttggcatgtttccacgagatccatgtgacgtgaaatgcatctgttcatttcaatagtgaaatagaaaaaaataaaataaacagtgcagggtatatttggtgagtcactgtggaacacagggccaaaataacttctgtgttgtcagtttattctatacaaccttattgttatgatgttagccttttcttataattcaaaaaaaatttattttaatagtgatgttttgttagcaaattaatacaaattcattgtagataaatcagaaaatacaaaataagaaaattaaaatctgctgtaacacacacccacacaaataccaatatctatattggtatgtgcatagtaggggcttaatatttatttgctaaatgaattaatatatattttacttacaaatatgagatcatactgtaatacttttataacatgctttagaaattaaaagacatcataaacatttttactgtgttattaagtattcttctttagcataattgtaatagttttcattattatgggacaagtaagttatctggaactcctgcaaaatttcttcagtagccaggaactgaatgcgagcacctcccagtaagactgatactgtggtgctgatatgatgaaatctgaacatgttcaacattttttgctgggatgtcatacatattctctgattactgagctagtaaatggaatctcagctgtcctgattgtgtgtaattctgtcatttctaccaccagatagagaccatcactgcttacatagataacgtgccattcacatccaggtgtactaatgtgagagagaatggccaaagatagcaatgtgcttggcacacccttgcacgccatcgtgatcctcagagtgaagtaagaatggctattgtcttccacaacatcttcaaggttgctgcaggggaagagctcctctgtcacaaggtgcctcatctgaagccactattaaagcgggtgtccatgctgaccagaaacaaagcacatttcacagacctattaacagttggaggcaggtgtttcctggttggtggacgtttcttctccacttagcaactcagggacacaaactgattttgccttctctttgtcagggcttcaaattcatcatctgcctccagtcagtgaaagaaaaatgagagcttggaggtggaacacctccttctttaaagctctgtcccagaaattgtattcattactagaactcagtcatgtgatctaactgcaagaaggctgggatatgtagtccaattgtgtacccaagaacagaaaatggtttgttagggaggggagaaacagcaaccattatctgaggttgcttaaatttggtcatattttgaatactttagtacatgctggcagtgctgtaaataagcaaaaatgaatccggcacccacattctgattgccaccaacttcgtgtaattttttaaaggtatataaaattcatgtgtcaatgcataaagatccattttaaattgataccataaaaaacaagtggaattgctgggtcaaatattcatacagaattctctggcttttcattaagtcgtgtctaattgaccctgagaaattgttcaa

SEQ ID NO: 15641 - RNA, 20402 nt, Homo sapiens
  source 1..20402: mol_type = other RNA
gctgggattacaggcatgagccactgtgcccagcctatttgtgagtactcttaaggcaatatgatttgcctaagttcaataaaaatcggctctcgttataacaggatacaattggaaacactggttgtattaccaaggctttgattaaaatgtcatatttgagaatgtgtagaatgcctggcttcaatggttctcagcattacactgaattaaaaattatcatttcctggcaggcccaggaaccttaaaactataggtaaaatctaaagtctaccttgacttagcttcttagcctcaaggaggtttttaaatctgagattactgtgaccatactactattcttgcagacaaaatctgataaagtttacaaatctgttttattctgaacatctttggtaaaaatcagggtaactttaagtttctgaagaaagctatatgtacctgttattagatcacagctctgtaccgttttgaaactcctgttatccacctgcagactggatttgctcctgaatcctcctaatttccttcaatatttggctatgactctctaagaaaaaaaactactcccatgctctgaggcctataagctaagatgtgattaatttttaaaggagcaagtctcatgctgatgtatgggtcacacaaaagttcaccataccaaccaatgccatagctagagacattcaaactgcaaaccaggacaaaaagttgatgatttcaggctgtagacatttttcctaagacatcagagcaagaattgtattacaatttgatttattcaattggttgcctgtaagcctaggttcagggctcaaaaccattatgcaaactgggattgtcacattactattaattttgtgtatttcctttttaaactttgtatctgttatttgccaaattttctgcagaaagaagtacaattcctaacagaataatgctagcccagcactttgaggggacaacaaaggactaaggaaaaaaaattggacttaataatagactccaggtggacttagcctaagtgccactcccttaaagcctccctgccctcaaaggtggctaaaagggttttaacactgacttttagttgccaatcactcctgccaatgcaggatgcaggaccagaccaataacccgggaaaggtctattctgtcaccaagggacaatcaaagcctaactacaagatgattcatcatagatactttcggaaaaacatcttcatcaagagagggaaaggtgaaagctgtcagaatcaagagtcatgtttccaaaagccctgacaaatggagccagggaagtccatgaagagagggattttacgcactacctcaaagacccagaagaaaccacgccagcttgcacaaacactattcgcaaccttacacagaaaatacttttgggacatctgcctagaagccgattgtccaaacccgaactggcagcatccttgttattaatccttgtagccaagaataattatttcaagacaattatataatctttatctgtcctttaaaaacctgtcttcctttaccttcctgaatacacacagtttactatggcatgcatattgccttcacaatgccctattcccaaataaacatcattttcttttagaaagcctctgttatttaggttgacagttattacacctgaaaactaaattctagctgatcaataaaattctttggttctactgtatacttttatttggggatatctgcttccaaacacactaaagtacagtatactcaattttaaatatagacagtatatttaaaaaaaacataaaaagtatgtcgaacatttttaatttcaaacaccaaacttaaatagactaataacacagatcttctgtggtccacaaatcatggcaaaaaactttgttttcatatgcccattatggcttgctgactggcttactgcattttagattttccttatgattttagtagctttctctaatggaatgtgctgtgagtgaagcttcaaacattttccattgaatatacacagacatacaaataaagactggaaaaaatatacaccagtcgttttctctggttgttggaatctgggtgattttttaaagtcccatccactgggctgccagtaaaagaccacaaaatatttttgtgtatttacaggaacgtgataatcaaaagttgttgtgggaccattcaagatgagcgtggggaagggaagcccatttaaacatatattcaaggaaaaatatattaagttacctgaacatttgggtagaaatactgagcactgctatggtctgtctcccaaactgtccctcaaatgtatgatgagattttatcttcattgtggtggtgttgagagctggggcctagtgggagatgtttggttcactgaggcagatgcttcatgaatggcttggtgctgctcttgcaatgagttctcactctctcaagactagattagtccccaggagtgggttgttaaaaagagacttgtttggttgttgtgaacaagtgggttgtttgcacgtctgcttcccctctgaccttctccatcaagctatgaagcagcagcaaagcccttgccaaaagccagggccatgcccttgaacttcccagcctgtagaactgtgagcatccttcataagtgaccctgcctcagctatcctgttatagtaacacaaaacagactaagacaggcacacaaaagctgaggactgctgtcgactccactttcaagggctaccaagcacagccacatcaccaaagagaacaattcctgacctccttggaagcagaaacttgactctccgggcaagataactgttgtctttttaaaatttcagtgtcaaagttaaaacatgccttgatcagtcaaccaaattactgctaaaccagtattgggaagcttcctaaagcactccaagctcctaaaaacaggcagcatgaagtaaagcagatagcatctttgcatttaagaagtcccagaaaggttttggaaatggcattaatgtaaatgttcacattaagagaaaacggtttccctgaattgagtgattctttctactttctagtgctgtacaggataggctcagcgtttggagagtgttaacttccagtcatgtgataatggccaggagcaaccacaatgattaacctttagatagaaaacacaatcctttgcttttgtcttccttatgtatattagattaggcttctactcaatgctctgtaagttaaaacatttcaaaccaaataggccactctattaagtcccagcttgagcattcttcagcttctccacattttccattgtttgctggcaaaccagtacagtaacctgttaaatacaaagcaagggtgtggtagattgactgcatttaaggctccaattcttcacccctcctatgttctctcccttggtctaataactctgtagtgcctttccacactgggtttagccatgtggcttgtttctggtgaatgctagttagcatgaagcatgcagacatgaaagggagttatgggattgggcttggctgttgttgccttctacaacctccacaaaaacatgcttgtttaatggaggataggaggcatgtggaaaaatgccaagtccttccaggtgaggccaactccctcatgaacgaggaaagactacaactgctccagagacatctagccgaaatcacttatctaattcataaactgtttattgctgcacaccactgggtttttgtggttgctacgagttacttttgcggcaataattgctccaatatgttctatgtgacatttctgagtttaacatcacatttacaaactttcttagagaaagatttgttattagcaaagaccttcagagtaacctttgcctggtattctagactgtgcagatttagccatctaatactgagtacccacttcaggctgaatgatctctcaagtgctctcatttagttctcataaccaccctaaaaactaacttcctcattttagggaactggaggaaatgaagaactttaaggtagactgatgaaaagatttatctaaagtcacataaattggcacaatcagggtccaaaccccaggcctccgattctgagtcaaactgcattttccattacatcggaaatgaccaaggattaaaattagcagaatgttattctgtccagccattaaaatccaaaaaaaaaatttgttcaaagtaggcaattgagttttcattctattatccaaggtaactgaagtatttgactgtacaggactgcttccttcaagtgttccatccttagcattcttgttaaaaatggcctttaagatattgctattcccagtcaagaaatacccagacaactaaagagactaaaatcatgtaaatcatccatttcccagttgaatcttaaaaaaaaatttatgctcaatacctctctccagccaatcactatgtaaattgtgaattaagacattattacttggtggcaataacggttagaaaaaaagcacatccctctccctctcccgtctccccccgtctcccactttctacggtctcccactttccaccgtctccctctgatgccgagccaaggctggactgtactgccgccatctcggctcactgcaacctccctgcctgattctcctgcctcagcctgccgagtgcctgggattgcagacgcgcgccgccacgcctgactggtttttgtattttttggtggagacggggtttcgccgtgttggccaggctggtctccagctcctgaccgcgcatgatctgcccgcctgggcctcccgaggtgctgggattgcagatggagtctcgctcactcagtgctcaatgttgcccaggctggagtgcagtggcacgatctcggctcgctacaacctccacctcccagccgcctgccttggcctcccaaagtgcggagattgcagcctctgcccggccgccaccccgtctgggaagtgaggagcatctctgcctggctgcccatcgtctgggatgtgaggagcccctcagcccggccgcccagtctgggaagtgaggagcgcctcttcccggccgcccatcgtctgagatgtggggagcgcctctgccccgccgccccgtctgggatgtgaggagtgtctctgcccgaccgccaccccgtctgggaggtgaggagcgtctctgcccggccgccccgtctgagaagtgaggagcccctccgcccagcaaccaccccgtccgggaagtaaggagcgtctccgcccagcagccgccccgtctgggagggaggtggggggcagcccctgctcggccagccgccccgtccgggaggtggggggcaacccccgcccggccagctgccccgttcgggaggtggggggcagcccccggccagcatccaccccgtccgggaggtgggggggcgcctctgcccagccgccccgtctgggaagtgaggagcccctctgcccggccgccaccctgtctgggaggtgtacccaacagctcattgagagcgggccatgatgacgatggcggttttgtcgaatagaaaagggggaaatgtggggaaaggaaagagagatcagattgttgctgtgtctgtgtagaaagaagtagacataggagactccattttgttctgtactaggaaaaattcttctgccttgggatgctgttaatctataaccttacccccaaccccgtgctctctgaaacatgtgctgtgtccactcagggttaaatggattaagggcggtgcaagatgtgctttgttaaacagatgcttgaaggcagcatgctcgttaagagtcatcaccactccttaatctcaagtacccagggacacaaacactgcagaaggccgcagggtcctctgcctaggaaaaccagagacccttgttcacatgtttatctgctgaccttccctccactattgtcctatgaccctgccacatccccctctccgagaaacacccaagaatgatcaataaatactaaaaaaaaaaaaaaaaaaaaaaaaaaagactttagttcaagttgagaccaaagactgtgctattatggggtggagaaaagtatcacaattttggtaatactaggcaagatgtaacctcaagtctccaggcagccccatgagcttccctgtgaatgagaacagaaaaagttcaggagccaccagaggatgttaaggaggcttcctagagaagacgtggcaatgcacctgatggagacgtttaatttcttcactacaaggaatttcaaacttatctaaaaggaaatagaatacaacaaagctcccttacccaatcccaacaaacaaccatcaatgtcctattcattcatacctccatctacttcctctgtcacatactattttgaagcaagtcttacccattgtattttacccataaatgtttcattctgtatctctaaaacattgtctctagacctcagcaaaaaaaaaaaagcacatccacttttacaatggtcacatacaaatggggaaagagtggatataaaaaatatgcacccaccttcaatcaaatgcgatcttttaaagaatataaacaagccagattcttaggtatctctcccttttgtaattttgattctgaaaaaatatttaaagtaatcaattaggtattctaaaagaaggcagttttctaggggtttatttaattataggggggttggggtagagagattaaaaacgggaagcagtgcataggcagtatgaagtagacactttggcaaataaaaactgcaccgtatgacatgtcacatagaaattgttagagactttgaatcctaaaatttagtttaccaaatgtagctttttatgttttatgttttaccaacaaataatttgtatgttaaatttaagcatctgaattccgaaatgataaagaacaggaaaataatgactaagctaacaaccaaactttcagagtataaaattttgtcagtggttttcattttagaattaaaaatttgaatttccctttgcctacaagtctaagtaacttgcagcagcaaattcccccactgacaacttcaaagcatagcaagaatccacagtggtttgcaggccactaattcttttacagatgaaagcattcaattatctctataaaattcaattccttagaatatgtgtttgtgattgacgatgtacatttttaaatgtggtgataacacgttattattcatgatttaaaagttgaaatgaagtagcttgtggttcttgggtaaaacagacactaataagttttttttcaatataaaagagcaacctagacattcctataaaacatttttattccaggtggtaagctggcttaaattttcacttttcagccaggcatgatggctcacgcctgtaattccagcactttgggaggccgaggcaggcaaatcatctgaggtcaggagttcaagaccagcctggcaaacatggtgaaaccctgtctccactaaaaatacaaaaagtagttgggcgtggtggtgtgtgcctgtaatcccagctactcaggaggctaaggcaggagaatcacttgaacccaggaggcgaggctgcagtgagccgagatcgccccactgcaccccagcctgggcaacagagcaagactctgtctccaaaaaaaaaaaaaaaaaattcgtttttctcacagcagcacatttctaaatggcaaaccatttagaagtgagtcatcatttgtattaaaatcttatttacatggtacttatgtagtttgatcaaatactgccacaatatagtttagaggcaagacctctcatgaagaaaaactttacaagatttaaaatcagagcaaatgaatttcttaagttcaagatacgtactctcaatggagaatcgctgttgggcagtggttaaggcctctgatttgctacttattagaaaaatccacatatatacaaaactctgctaaaattccaatggcttctctagatgaatcatctttggctgtgagcaaaaaagttaactaagtttcacttaatacacacacacacactagggtttatatgtagcaacttcctcatcctcattccacaggtagcccgttcttggctgggttatggcttgtaatctcagaaccactgcccccaaatgactgctcagaagcacaatctcactgcaaactatggaacccaaactatacagctatccttggcttttaactccaagctatctaggccttgtgattatatgtgggcttcatagcagaacctaccaggcttgtggttatcaattttctgctcaccatataagcagtagctcaataacaccgtccagttttcatgtatatccagacacacaggtgagagttctgttccaagatctcattttgaccttcttcaaaggtcttctccatctctccaaattgaatgtattcttcaaccctgggcttactgtattctgcccatcttcttcctggaccaaactgttcagaagttaacttctttttcctgtcatcacatctctttcctaaactactttagaacttaaataattttattttcacataacatttagaaaggtgcagaggcagccaacaaaactattgaagacagactgtaaaaactggcaaatccccatctcaaattccatttattctataaccaataaagtcatgcagtttggacgggagcacagtaatacattctgttctcatgtagcttcctaagtatgcttagtctattgttcatttatcactgaatctgttatctgctaagtctgattcaatgttcttgccttctattaatgtgattttaagaattactgcatgtctcactatggcaaaatagcatgacatttgttttacaaaatcagttaaaccaattctacaaatatttccatacctatttattgcagcaaaagataatttttatgtgtaaattagctttttgggtttttctattcctttatttgtaaacttataatttttaggttgggcttactattttgatgagaagggtgaatctgtcaaagggtaagctggataactgtatgttgcaaacatgttcctgaacattcttcacccaaacttagacaaacctggagcttaaaataattacattggatgacatcagtttgatactgatgcctgcttcctgcactaagaggctttcaatctattttgaagagggaaaaacagaatatgccaagtggggagacagcccaaacatagaccttaatacttctctcatactcttcagccatttgatgaacatgtggaattatggatgctagggccattataaaaatctcctgatacagaacagtgtcactacttcaagctaagcagtgacaggcaaagccaggctgaggtgacaatgtagaaggatctcgagtcagccctcaatgttgttgttcaatgttgggaagtcccttttagattatttatacagtggcaggtggtagcaattacagtaaattttcttgggtttcttcctaataaaaaagtgttgataaaactacaccagtcccaaggctattcaatgccacgtaaaatagtgtattttagcatttgaggtccctttttgttgcatactaaagcatgtttaaaatggtttgcagaaaacagtctgctaaccagtactgattcatccacagaactgaattcttgcaaggcacaaaggaagtgtggctgacctaaatatttctcatttttaaaattattcatactgattatatgagattatatcttatctagtatttttcaatggagccttaaaaatgttattttgttaaaagtatatttcagcaaatttcaactttgaagatgtttttgtttacagcatagatcttatgtattagagcgctaatgtagcataggcaaactctgaaataaataaaaatgtataaatagcactgtgcagtgtgtggtgtgcgcctgttgtggggttatattaagtagtataaatttatctcccggggggataggataatcttttatgtaacaccaaattaaaaaaacaaaaacatgtactcttaaaatcatatgtccatatgtgaaatacaatcactttttttggtttccatataatttagggagtgaacaccaaaatgtaatcccatataaaaaaagatcagtttaaataaaaattaaaacaattaaaaattagtcccatagtaacatggtaaacaactcaaatggctttcttttaatgctaggaaaactgtccacctttcaacggtgacagggctgttaacacaggtaagagcaaacaaggtaaaaagtgaaagcacatacagatgatgcacacaaatatatataaaaattgaccagaaatcacaggacatgtaagcaatgttttcttaagcagaactttttttgtactttaaatagactaaaatatttggtgtaggtgggagaaagacatcagtattcaacaattttaacttgaaaaccagctgtaataaagcctcagctcattgtttaataaaaataaaaaaggaaccacatcgtacttttgacaatcatagaacgaaagctcacaaagaacacatttaatatctccatcacagtgcaccaaggatgcagccactaaggacttccagagggaaacaagaacagggtctgcatccatcatattgcattacaaagttaatgccatcagagaaaaaaaatctcacctcacgtgctcaatgttctagctggtaagcaccttatgagtatgaggctacaattgagagaaactgctcagtctgcatcaggacacccaattccttcacttgccattggctgatgcatttaatcattttaacacaacattcacggaaaaatgttaacaacacattctggcttctcgagcagaacagactgggaaatgcagtagacgccagagcatcaaaggccatgtatttcctcacaagaaaagaaatctgcaacaattggtttccttttactatgaaaaatgtaaatttcagattaagtttaaccccataaggacgcatgatttgtacttacatatacacataggttcagaagaacttagctatctagttggcctcttctctgttccattataacatcagttaccttagctggatcactaagtgtgagtctcaccaccatactggtaccttcagctattacctgtgttataaatctcatgttccattcaaagtactaaatgactggatggcacatatcccaataagtatcagaaatgttgacagccatagtgcagctgagtttagaagcaactatgacaacatagggaagtaaggataaatcacaagaacacctaaggtggtcagctccttctggtgtgcctgggacttgttttgagtttagcaaaaactttacaagattaaaaatcagagcaaatgaatttcttaagttcaagatatgtactctcaatggagaatcgcttttgggcagtggttaaggcctctgatgtgctacttatcagaaaaatccacatatatacaaaactctgctaaaagttttgtatccagggaaagtcccgcatccagggaaaccctcaatcccaggcactttagggcagctggtcaccctgagaacactacccactcgttccttaatatcactagagaaaaggtaagaactttcaagggcataacctttaagggcatcagtccccaaaatatttttacatcactagctaatggctagttcctctaagcttgctaaaaggctaggaagtccagaaataccttaaacgtgttaactttaagaagagttggtagtaatcaagcaaattagtgagcagtgtataaaagctcactcttgaaatctgttttcagacaaatcttctaaaggttcttctagctttgtccagttatatggtattttactgtattctctttttgcaattaatccagttttgtatgtcttttctttcttttttaggtgaaaatattctatgccaactgttttccacagtcctgcattatatattaaaacaaaggctgccagctggagacacagccctccgattacaaaggcccagaatgttacttttaactgtgctccaccaggaggtctggccttgggaaaagatggcgaaaggaatattctcagatatgaacattttttattctgcctacaatgctgtgatctagttcaacaactgcagaactgttctcatcttaatcgctgtagtttttctttctttactcttttgtataaaaggttagtgtcacagcttcactatcactaataaaaagatacaaatatgcctttcaagtcagggttggaaaagcaaaactgaggtgtgaggttacactggtctaagaaagtaccaatttgggttctatattttgtcaaacagttgggtttttaaaaaaattcaaaactcatgcatgttacctacttgtcatgtgtgaattatttctcacaattttaattaatctgtgtgtatattagttatataaagcaatggatttccacattcttaaagcaggaacctatattcaccagaaaaggatcctcctgtttctcatcaaattttttttcagctcgaacaatccaagattgggaatagtaagagtggcaaacaaatgttttcttagggacttactgagaaaagaaaaaacttactgggagaacagagacttagtaaaatttctattgctacagacaaatgctaaaaaccagctttataataacagcattataaaggatagaacttaatatagaaccagaaatatggcaagttacctagtgattaacattgtaaaatagtcaaaaactttaaagccacagagaaaggaaaacaattatgaaatggaaaatatataatatttaagtacttttataattctaaaacttcacttttgtccttaaatcaatatattacggatttcattgttcaataaattaccatctttaattaaaaataagtaaatcaaagagcatatttggagaaactaagagctgttaactgtttggagggtaaaagaatacttttctcgaaatttttttgaagaaaaatctaaaagccctctatgttgagttaatacaccttctgacccccatcatcagtggcattattcttccaagggactcttatatctaagcaatggtgaagttctggattcattatggatctcatggcaccaaaccaactggcactgaagttaagttaatatactccagcgagatcacctgtgggtcaaggatggcccagagaatcttggaaaatccatttatattgagcaaagatctgaatcaccttcaatcaggctgtaagatactagaaaatttgaccttgtagtagtatttcccagggtaacttaagcagcaaccttgcaccagaagaagaattaaagagggagcaatctagtattatcaacaacaacaaagttaaccctaagttagtacatcccagaatctgctggatgtataataatttagtaacggggtatatggcagagctttctttgatgttaacaaattttggctgtgattcttagttaccaagttgccaaaaaatggtatattaaatgaactgccaaatggcagattaagaaaattaatgtactccaatggtctgtccatgaaaggaaaatgtacacagacaaattaagaacattttaccaggatctgagatttaaacaatggaacaattgttttaactgttagaatgaccccaactgttaagtttgtctatgagtgtatatgtatatataaattcatacacatatattatttatttccttcttaaaaagactgaggcagttctgctatatatagttagctacaatattcaagataaaacagttcctactcaaaaaattacatgaacacacgagataagttcttatcgtaaatgctatcatgaggctatctagtatagctcatatttcctggttgtaaggctcaaaacacaggaattccactccaagagataatttgcccctcaatccctacaaagtgtagtctaaacaaacaaaatggtaataaaaaattgaaaaggaagatataaaaagaactcaatagcaggattctgactacctctggagaccacacactatcattattctgactgtcttaaatacaacaatccaatatgccccaagatggaaatctggtatcgtagggaaaacattggctgcaactgtcagaaaagttcataatcttaaacataatttatgccatttgccagtcacaaagacatttactgaacagaatttttgagccatttgtaaaattaaaatgattgatcaatttgaatagcaaccttcatgatgaagaaattaggactctaggtatgaaaagcatgttccttttttgttaataagttcaaaggagagaaacattctgatatatgcagataaaaatatggctaggctgggcgcggtggctcatgcctgtaatcccagcactttgggaagccgaggtggacagatcacgaggtcaggagatcgagaccatcctggccaacacggtgaaaccccgtctctactaaaaatacaaaaaattagccgagtgtggtggtgggcgcctgtagtcccagctacttgggaggctgaggcagaagcatggcgtgaacccgggaggcggagcttgcagtgaaccaagatcgcaccactgcactccaggttgggcaacagagcgagactccctctcaaaaaaaaaaaaaaaaaacaaaaaacaaggctaacaagaaagaggataaccagcaagtaccacctggatgtgtgttgtcaggtagaaaggaagaataaaattcaggcaatgaatataatagatttagcaaagtaaagcatatgaaaggaagaaatgtttgatatgtctaagtatcaatgccttcgatcagagtaagaaaaaagtattcattgttcatgtccacagactagatatctaaagagatacttggtgggcaggggcttgggagggaaggcgcaaattggaatgttcagcttttaaagtaaagactgtacatgaagacatattttatgtacagtgaagattgtcttgtgttactttatatcccaacataaacctacgccaccctcagacgaagagggtatctaacactgaataaatgctgaacctatttagtagttaaagaaaaaagagaaggatcttaaaggtatatatgggaagcttttaagaggtagagaaaccaactgggtatatattttcttttatttgatttcaactagcaagagactaagactgatgtttgtttgtttgttttaccttcaaagtcttagtcttaaattgacaagggcacaaaaaaagtgaaattaaaataattttaacaaaagggaaagcatttgacagtgtttaaaagacagacaaatcaagcaaaactcaatgtggcttaaggtaaaaaatacaactaggtattaaacaatttgtaaaaacttacaaagaaaatttagctttcaagaaaaattaggcagatttccttctgccaaagtgacaggtcctgaggaaaaaaaacacaacctctacaagaccaagcacagctcaagggtcagggccccgtcctagtcatctttttattattcaatatccatcacagtggctgggcaaacaacaggcatcaataaatgtttactaactgaatgtgtattataaggtataatcggtataactgatatagctcaaatctaatcatgaaagcttctttaaagtaggataaaaagagcacaatcagcggtattccagaaggtaggcctaaatccagttatatttttctaatcgttgaccagtggttataaagactttctgagcttctttttaaagcaatgaaactctttccaaaagaaaccccatgcagttcttcagtacagaataaatatgccactaagtcagtgagaactccaacagcctcccctaagccagcccccaaggtgtctctgtggaacctactggaaaaaatattactcatcttagaaatgtgatagaaagcatggccattcggttctcaggtcatcattcctagaaaattaacagtattgtgaagaataaatcctaagtaatgttgctaatttaaataaagacaaaaattcaacaaagaggggattctatcacttagaaaaatgaaaaccacacctataaatggggggaggggcagaaaacaaaaaaaaaatcaggccacagtagataaaatacaaaaaacatcatctcgttaaaaagcatcaaacacattcacacaaatgtaattacaaccaggaagtaaactgctcaacaggtataactgctcaataggtgttttcaaagagttgagtcccaatttcatactgtacagaaaaatcgcatcagaactgtagagatgcgctccactactgaaacagcatagtaggcactgcttgacctaacacagtaatgcaagagtaaccaccaagatcaggaccttctaccactttcagagttgttttctgcccctacaactgttccctaacaccattacaagttctcaagtaagaaaaagaagggcagaggctccactgagtatctcctacaggcctgatagtggtattacctaggacatttactctgctcacaagatgggtagtggaagacataattactggacagcacaaagtctggaagcaagcagcagggcactaaaacagtgagagcttacacaacaaaagcttgttaaattaagtagtactgatgtggtgcaaatgaaatttttacagcaaaggttgaggaaggagatatgttagtgagaatcacatgaagcagactatcacaaaataaggccaccttcaaaatgttatgaactgtagaaccattctgatcttcaagtttggatttgtatagaggtttctgtataaagcattaatacctaatcaggagtttcctttagtgtgaacctttttgcatttgatgctattctctttgccaggaatgcttatctcccctggctcctcacttggcttgcttctttaatgtcaggtgttagctcatgcatcctttccttagaggctttccttgatgtcctacctgaagcatcccatctgttattctccagtacagtaccctgtttatctccttcatagacaagtaagataattaagggttagtgtaactgctgtctcagcaaaggcaggaactgtagttgtcttgttcacctttacccaaagactaagaaaagttcctggtacaaacaggtgaacaataaatatttgttgaatgaataaaaaattactataccaaatttacatgaacacatacatatacacacaaatataggaaaatggggagtacccaatagaaaaccaccaaatgttgaaagtattgaaaatgatacctatagagacaggtggatatgatttcaaagaacaagtaccaaagacagcttcaaaaatatgaaaatttatgaaaagacgaccaggagtggttattttccatttctactaagatgcaaacaagaagaaatgtttaaactgcaatgagtcaacatcagacataataattatttgctgcagaatgaactagcaacagagtttcggaaatctcctctcactacagagcatgaaatattgtcaatcacaaaaccaggatcagttaagaacagctcagactgcaggtaacttataagctaaaaaacttgctaaataaatggcttttcccccaatttttaaaattctgaattcataattatgtgtagaataacaatcaatttataaactgaatacaacatactttaaaaacagatggcccatatctgctgatcctacctcagcatcacttttctaggtattttgcagaaacaattacatttacaaaaggcccatttcataatgcaatctggttactaaaccaaatcaaactactcgaagagcagaaggtctgctgttgaaatattgtaaaatacctttggaaaaacggtatttatagattagcttttttaaaaagggataaatatgtggaagtaattctagcatatccctgaaaataattatactgccacctatgcattttttatgaggtggaaggataaatcaacagactgctagattatacaagccaattattcctgttgaaatttgggcataagacaaagggactttctccatatgaattcttactgtatcccagaattaactggtgccagcagtatcaatgcaactattactggtgatgatgtcatgttatgctgttttgattatgaggacaaaaatgggaatggaaaaaagaggcttggaaaggttttcagtatggtttccttataataagatttagcagttaaaaaaaaaaacaaaaaaaaacaaaaaaccacaaaaagaatgactgtttaagccccactgaacacattaaggtcaaggatttcaaaagttaatccacttttcttcccccaagagtttatttttggtaaaaggcagaaaaattagtttttctacaggaaaatctgcttctaaataatttgaaaatcttgatatatattatatattaaaaaagacacacaaaaataacagagaagtgggaataacagattaggtactgcaactttataaaggtttgcctagatcaagaagcagcgcacacacacacctcatctatgcaaactaaaaatgtatataaacagcacaatactgtgatactggatcatgatacattacctgtacacataactactactgttattaataaacctttgggacactcagttttatgcccaataagacatcattaagtctttaaaatcttctcttcctctttaatgggagagtatttctagacactaattttcccatctaatattcaaatataggaaacagattccacaaggtgctttaattgatgagacctcaagtgctgttttctctcttgaacttttggatagtaaacagtccatagggaccacacacaatgctatgacagaagagttgttacattaagtcttttcatgggacttgattggtgaagctttatgacatgcttgagcaacgcactgaaggggatcccatctgagttaatactttgtccaaccactgtagaggtccattcagatgaagttcaatccagcaaggagtacttgttaccgtctgccttcggtattctgctccccaccctttcacaaaactcattcttatggtgcacattctagttagctgatagacggcttcaaaaccctgattaacagactgagccagaagagcagcaaattcctggttgttgaagatcttcagattacagcctggtggaattttacacactgttgcagggtgccagccatatctctgattacaattggggctctgcacaaagattgcactatcacttaggcactcagcaaaaacttccccacctatgtagtataagcgcactcctcttcctatatgccttcttgtcatttctaccgtggcatttcggttaacattggagagtaaacctaagcagaacctctctgaatttgatgggtctgtaaagccatctacagtgagtgagggctgtgatgcatggaaggtttctccaaccctctgatttaattcataatatgctatcgaacaccaaaatgcaggttctgagtaagtaactggctgtaaatccaagctatgattaacaggggaaagagtagtaggagatagttctgctggagagcctgtgtccatactttgattcaactgttggtcacttgtttctccatcttcactgatatatccaggaggtggcgtttctggaatataattactctgtggctcaattcctgctgggaagttagtgttttctggaatggagtgagtatagtcatccagaggcggaagttctgttaggatctcggtgtgtcggggcactaatactggaggcaaaactggtgtctcaactctctgatagtggtaagggtttacacatacttcatcctttttaagattaaaagcatattcgcagttttcaattgccttgagttcatgatgactgtgaagatcaggccagcgccataatcggcaatatataacatgtggcaatccttttcgatgggatacctggagacgaccatcaagagacctggtttgttcagagaagctgtaaaggcctgttgtatcccactgatctatcgtatttggtgtactcagtccccaaatttcagagcaagtgcttggtatggtaacacatttagtattacagttttgagtggtgatggctttctcaagctcatctaatcgtcctgttttctttagcttcttcaccagacttttcactgctttctcacaccacttttcttcctgcccattctgctctcctccgcctgctcctccagacccaccagctgacttcttccatcccagcagtctcttcacaactggcggcgtgaatggcaagatggacgacatgttcttaccaaaggcagcaagccacgctaggaaaacagcctcttgtatcgaacctcccggcggctggcgggctgctggctggcgagctgcttctccgccgccgcggccgcgcgggtagacccgcct

SEQ ID NO: 15642 - RNA, 20628 nt, Homo sapiens
  source 1..20628: mol_type = other RNA
gctgggattacaggcatgagccactgtgcccagcctatttgtgagtactcttaaggcaatatgatttgcctaagttcaataaaaatcggctctcgttataacaggatacaattggaaacactggttgtattaccaaggctttgattaaaatgtcatatttgagaatgtgtagaatgcctggcttcaatggttctcagcattacactgaattaaaaattatcatttcctggcaggcccaggaaccttaaaactataggtaaaatctaaagtctaccttgacttagcttcttagcctcaaggaggtttttaaatctgagattactgtgaccatactactattcttgcagacaaaatctgataaagtttacaaatctgttttattctgaacatctttggtaaaaatcagggtaactttaagtttctgaagaaagctatatgtacctgttattagatcacagctctgtaccgttttgaaactcctgttatccacctgcagactggatttgctcctgaatcctcctaatttccttcaatatttggctatgactctctaagaaaaaaaactactcccatgctctgaggcctataagctaagatgtgattaatttttaaaggagcaagtctcatgctgatgtatgggtcacacaaaagttcaccataccaaccaatgccatagctagagacattcaaactgcaaaccaggacaaaaagttgatgatttcaggctgtagacatttttcctaagacatcagagcaagaattgtattacaatttgatttattcaattggttgcctgtaagcctaggttcagggctcaaaaccattatgcaaactgggattgtcacattactattaattttgtgtatttcctttttaaactttgtatctgttatttgccaaattttctgcagaaagaagtacaattcctaacagaataatgctagcccagcactttgaggggacaacaaaggactaaggaaaaaaaattggacttaataatagactccaggtggacttagcctaagtgccactcccttaaagcctccctgccctcaaaggtggctaaaagggttttaacactgacttttagttgccaatcactcctgccaatgcaggatgcaggaccagaccaataacccgggaaaggtctattctgtcaccaagggacaatcaaagcctaactacaagatgattcatcatagatactttcggaaaaacatcttcatcaagagagggaaaggtgaaagctgtcagaatcaagagtcatgtttccaaaagccctgacaaatggagccagggaagtccatgaagagagggattttacgcactacctcaaagacccagaagaaaccacgccagcttgcacaaacactattcgcaaccttacacagaaaatacttttgggacatctgcctagaagccgattgtccaaacccgaactggcagcatccttgttattaatccttgtagccaagaataattatttcaagacaattatataatctttatctgtcctttaaaaacctgtcttcctttaccttcctgaatacacacagtttactatggcatgcatattgccttcacaatgccctattcccaaataaacatcattttcttttagaaagcctctgttatttaggttgacagttattacacctgaaaactaaattctagctgatcaataaaattctttggttctactgtatacttttatttggggatatctgcttccaaacacactaaagtacagtatactcaattttaaatatagacagtatatttaaaaaaaacataaaaagtatgtcgaacatttttaatttcaaacaccaaacttaaatagactaataacacagatcttctgtggtccacaaatcatggcaaaaaactttgttttcatatgcccattatggcttgctgactggcttactgcattttagattttccttatgattttagtagctttctctaatggaatgtgctgtgagtgaagcttcaaacattttccattgaatatacacagacatacaaataaagactggaaaaaatatacaccagtcgttttctctggttgttggaatctgggtgattttttaaagtcccatccactgggctgccagtaaaagaccacaaaatatttttgtgtatttacaggaacgtgataatcaaaagttgttgtgggaccattcaagatgagcgtggggaagggaagcccatttaaacatatattcaaggaaaaatatattaagttacctgaacatttgggtagaaatactgagcactgctatggtctgtctcccaaactgtccctcaaatgtatgatgagattttatcttcattgtggtggtgttgagagctggggcctagtgggagatgtttggttcactgaggcagatgcttcatgaatggcttggtgctgctcttgcaatgagttctcactctctcaagactagattagtccccaggagtgggttgttaaaaagagacttgtttggttgttgtgaacaagtgggttgtttgcacgtctgcttcccctctgaccttctccatcaagctatgaagcagcagcaaagcccttgccaaaagccagggccatgcccttgaacttcccagcctgtagaactgtgagcatccttcataagtgaccctgcctcagctatcctgttatagtaacacaaaacagactaagacaggcacacaaaagctgaggactgctgtcgactccactttcaagggctaccaagcacagccacatcaccaaagagaacaattcctgacctccttggaagcagaaacttgactctccgggcaagataactgttgtctttttaaaatttcagtgtcaaagttaaaacatgccttgatcagtcaaccaaattactgctaaaccagtattgggaagcttcctaaagcactccaagctcctaaaaacaggcagcatgaagtaaagcagatagcatctttgcatttaagaagtcccagaaaggttttggaaatggcattaatgtaaatgttcacattaagagaaaacggtttccctgaattgagtgattctttctactttctagtgctgtacaggataggctcagcgtttggagagtgttaacttccagtcatgtgataatggccaggagcaaccacaatgattaacctttagatagaaaacacaatcctttgcttttgtcttccttatgtatattagattaggcttctactcaatgctctgtaagttaaaacatttcaaaccaaataggccactctattaagtcccagcttgagcattcttcagcttctccacattttccattgtttgctggcaaaccagtacagtaacctgttaaatacaaagcaagggtgtggtagattgactgcatttaaggctccaattcttcacccctcctatgttctctcccttggtctaataactctgtagtgcctttccacactgggtttagccatgtggcttgtttctggtgaatgctagttagcatgaagcatgcagacatgaaagggagttatgggattgggcttggctgttgttgccttctacaacctccacaaaaacatgcttgtttaatggaggataggaggcatgtggaaaaatgccaagtccttccaggtgaggccaactccctcatgaacgaggaaagactacaactgctccagagacatctagccgaaatcacttatctaattcataaactgtttattgctgcacaccactgggtttttgtggttgctacgagttacttttgcggcaataattgctccaatatgttctatgtgacatttctgagtttaacatcacatttacaaactttcttagagaaagatttgttattagcaaagaccttcagagtaacctttgcctggtattctagactgtgcagatttagccatctaatactgagtacccacttcaggctgaatgatctctcaagtgctctcatttagttctcataaccaccctaaaaactaacttcctcattttagggaactggaggaaatgaagaactttaaggtagactgatgaaaagatttatctaaagtcacataaattggcacaatcagggtccaaaccccaggcctccgattctgagtcaaactgcattttccattacatcggaaatgaccaaggattaaaattagcagaatgttattctgtccagccattaaaatccaaaaaaaaaatttgttcaaagtaggcaattgagttttcattctattatccaaggtaactgaagtatttgactgtacaggactgcttccttcaagtgttccatccttagcattcttgttaaaaatggcctttaagatattgctattcccagtcaagaaatacccagacaactaaagagactaaaatcatgtaaatcatccatttcccagttgaatcttaaaaaaaaatttatgctcaatacctctctccagccaatcactatgtaaattgtgaattaagacattattacttggtggcaataacggttagaaaaaaagcacatccctctccctctcccgtctccccccgtctcccactttctacggtctcccactttccaccgtctccctctgatgccgagccaaggctggactgtactgccgccatctcggctcactgcaacctccctgcctgattctcctgcctcagcctgccgagtgcctgggattgcagacgcgcgccgccacgcctgactggtttttgtattttttggtggagacggggtttcgccgtgttggccaggctggtctccagctcctgaccgcgcatgatctgcccgcctgggcctcccgaggtgctgggattgcagatggagtctcgctcactcagtgctcaatgttgcccaggctggagtgcagtggcacgatctcggctcgctacaacctccacctcccagccgcctgccttggcctcccaaagtgcggagattgcagcctctgcccggccgccaccccgtctgggaagtgaggagcatctctgcctggctgcccatcgtctgggatgtgaggagcccctcagcccggccgcccagtctgggaagtgaggagcgcctcttcccggccgcccatcgtctgagatgtggggagcgcctctgccccgccgccccgtctgggatgtgaggagtgtctctgcccgaccgccaccccgtctgggaggtgaggagcgtctctgcccggccgccccgtctgagaagtgaggagcccctccgcccagcaaccaccccgtccgggaagtaaggagcgtctccgcccagcagccgccccgtctgggagggaggtggggggcagcccctgctcggccagccgccccgtccgggaggtggggggcaacccccgcccggccagctgccccgttcgggaggtggggggcagcccccggccagcatccaccccgtccgggaggtgggggggcgcctctgcccagccgccccgtctgggaagtgaggagcccctctgcccggccgccaccctgtctgggaggtgtacccaacagctcattgagagcgggccatgatgacgatggcggttttgtcgaatagaaaagggggaaatgtggggaaaggaaagagagatcagattgttgctgtgtctgtgtagaaagaagtagacataggagactccattttgttctgtactaggaaaaattcttctgccttgggatgctgttaatctataaccttacccccaaccccgtgctctctgaaacatgtgctgtgtccactcagggttaaatggattaagggcggtgcaagatgtgctttgttaaacagatgcttgaaggcagcatgctcgttaagagtcatcaccactccttaatctcaagtacccagggacacaaacactgcagaaggccgcagggtcctctgcctaggaaaaccagagacccttgttcacatgtttatctgctgaccttccctccactattgtcctatgaccctgccacatccccctctccgagaaacacccaagaatgatcaataaatactaaaaaaaaaaaaaaaaaaaaaaaaaaagactttagttcaagttgagaccaaagactgtgctattatggggtggagaaaagtatcacaattttggtaatactaggcaagatgtaacctcaagtctccaggcagccccatgagcttccctgtgaatgagaacagaaaaagttcaggagccaccagaggatgttaaggaggcttcctagagaagacgtggcaatgcacctgatggagacgtttaatttcttcactacaaggaatttcaaacttatctaaaaggaaatagaatacaacaaagctcccttacccaatcccaacaaacaaccatcaatgtcctattcattcatacctccatctacttcctctgtcacatactattttgaagcaagtcttacccattgtattttacccataaatgtttcattctgtatctctaaaacattgtctctagacctcagcaaaaaaaaaaaagcacatccacttttacaatggtcacatacaaatggggaaagagtggatataaaaaatatgcacccaccttcaatcaaatgcgatcttttaaagaatataaacaagccagattcttaggtatctctcccttttgtaattttgattctgaaaaaatatttaaagtaatcaattaggtattctaaaagaaggcagttttctaggggtttatttaattataggggggttggggtagagagattaaaaacgggaagcagtgcataggcagtatgaagtagacactttggcaaataaaaactgcaccgtatgacatgtcacatagaaattgttagagactttgaatcctaaaatttagtttaccaaatgtagctttttatgttttatgttttaccaacaaataatttgtatgttaaatttaagcatctgaattccgaaatgataaagaacaggaaaataatgactaagctaacaaccaaactttcagagtataaaattttgtcagtggttttcattttagaattaaaaatttgaatttccctttgcctacaagtctaagtaacttgcagcagcaaattcccccactgacaacttcaaagcatagcaagaatccacagtggtttgcaggccactaattcttttacagatgaaagcattcaattatctctataaaattcaattccttagaatatgtgtttgtgattgacgatgtacatttttaaatgtggtgataacacgttattattcatgatttaaaagttgaaatgaagtagcttgtggttcttgggtaaaacagacactaataagttttttttcaatataaaagagcaacctagacattcctataaaacatttttattccaggtggtaagctggcttaaattttcacttttcagccaggcatgatggctcacgcctgtaattccagcactttgggaggccgaggcaggcaaatcatctgaggtcaggagttcaagaccagcctggcaaacatggtgaaaccctgtctccactaaaaatacaaaaagtagttgggcgtggtggtgtgtgcctgtaatcccagctactcaggaggctaaggcaggagaatcacttgaacccaggaggcgaggctgcagtgagccgagatcgccccactgcaccccagcctgggcaacagagcaagactctgtctccaaaaaaaaaaaaaaaaaattcgtttttctcacagcagcacatttctaaatggcaaaccatttagaagtgagtcatcatttgtattaaaatcttatttacatggtacttatgtagtttgatcaaatactgccacaatatagtttagaggcaagacctctcatgaagaaaaactttacaagatttaaaatcagagcaaatgaatttcttaagttcaagatacgtactctcaatggagaatcgctgttgggcagtggttaaggcctctgatttgctacttattagaaaaatccacatatatacaaaactctgctaaaattccaatggcttctctagatgaatcatctttggctgtgagcaaaaaagttaactaagtttcacttaatacacacacacacactagggtttatatgtagcaacttcctcatcctcattccacaggtagcccgttcttggctgggttatggcttgtaatctcagaaccactgcccccaaatgactgctcagaagcacaatctcactgcaaactatggaacccaaactatacagctatccttggcttttaactccaagctatctaggccttgtgattatatgtgggcttcatagcagaacctaccaggcttgtggttatcaattttctgctcaccatataagcagtagctcaataacaccgtccagttttcatgtatatccagacacacaggtgagagttctgttccaagatctcattttgaccttcttcaaaggtcttctccatctctccaaattgaatgtattcttcaaccctgggcttactgtattctgcccatcttcttcctggaccaaactgttcagaagttaacttctttttcctgtcatcacatctctttcctaaactactttagaacttaaataattttattttcacataacatttagaaaggtgcagaggcagccaacaaaactattgaagacagactgtaaaaactggcaaatccccatctcaaattccatttattctataaccaataaagtcatgcagtttggacgggagcacagtaatacattctgttctcatgtagcttcctaagtatgcttagtctattgttcatttatcactgaatctgttatctgctaagtctgattcaatgttcttgccttctattaatgtgattttaagaattactgcatgtctcactatggcaaaatagcatgacatttgttttacaaaatcagttaaaccaattctacaaatatttccatacctatttattgcagcaaaagataatttttatgtgtaaattagctttttgggtttttctattcctttatttgtaaacttataatttttaggttgggcttactattttgatgagaagggtgaatctgtcaaagggtaagctggataactgtatgttgcaaacatgttcctgaacattcttcacccaaacttagacaaacctggagcttaaaataattacattggatgacatcagtttgatactgatgcctgcttcctgcactaagaggctttcaatctattttgaagagggaaaaacagaatatgccaagtggggagacagcccaaacatagaccttaatacttctctcatactcttcagccatttgatgaacatgtggaattatggatgctagggccattataaaaatctcctgatacagaacagtgtcactacttcaagctaagcagtgacaggcaaagccaggctgaggtgacaatgtagaaggatctcgagtcagccctcaatgttgttgttcaatgttgggaagtcccttttagattatttatacagtggcaggtggtagcaattacagtaaattttcttgggtttcttcctaataaaaaagtgttgataaaactacaccagtcccaaggctattcaatgccacgtaaaatagtgtattttagcatttgaggtccctttttgttgcatactaaagcatgtttaaaatggtttgcagaaaacagtctgctaaccagtactgattcatccacagaactgaattcttgcaaggcacaaaggaagtgtggctgacctaaatatttctcatttttaaaattattcatactgattatatgagattatatcttatctagtatttttcaatggagccttaaaaatgttattttgttaaaagtatatttcagcaaatttcaactttgaagatgtttttgtttacagcatagatcttatgtattagagcgctaatgtagcataggcaaactctgaaataaataaaaatgtataaatagcactgtgcagtgtgtggtgtgcgcctgttgtggggttatattaagtagtataaatttatctcccggggggataggataatcttttatgtaacaccaaattaaaaaaacaaaaacatgtactcttaaaatcatatgtccatatgtgaaatacaatcactttttttggtttccatataatttagggagtgaacaccaaaatgtaatcccatataaaaaaagatcagtttaaataaaaattaaaacaattaaaaattagtcccatagtaacatggtaaacaactcaaatggctttcttttaatgctaggaaaactgtccacctttcaacggtgacagggctgttaacacaggtaagagcaaacaaggtaaaaagtgaaagcacatacagatgatgcacacaaatatatataaaaattgaccagaaatcacaggacatgtaagcaatgttttcttaagcagaactttttttgtactttaaatagactaaaatatttggtgtaggtgggagaaagacatcagtattcaacaattttaacttgaaaaccagctgtaataaagcctcagctcattgtttaataaaaataaaaaaggaaccacatcgtacttttgacaatcatagaacgaaagctcacaaagaacacatttaatatctccatcacagtgcaccaaggatgcagccactaaggacttccagagggaaacaagaacagggtctgcatccatcatattgcattacaaagttaatgccatcagagaaaaaaaatctcacctcacgtgctcaatgttctagctggtaagcaccttatgagtatgaggctacaattgagagaaactgctcagtctgcatcaggacacccaattccttcacttgccattggctgatgcatttaatcattttaacacaacattcacggaaaaatgttaacaacacattctggcttctcgagcagaacagactgggaaatgcagtagacgccagagcatcaaaggccatgtatttcctcacaagaaaagaaatctgcaacaattggtttccttttactatgaaaaatgtaaatttcagattaagtttaaccccataaggacgcatgatttgtacttacatatacacataggttcagaagaacttagctatctagttggcctcttctctgttccattataacatcagttaccttagctggatcactaagtgtgagtctcaccaccatactggtaccttcagctattacctgtgttataaatctcatgttccattcaaagtactaaatgactggatggcacatatcccaataagtatcagaaatgttgacagccatagtgcagctgagtttagaagcaactatgacaacatagggaagtaaggataaatcacaagaacacctaaggtggtcagctccttctggtgtgcctgggacttgttttgagtttagcaaaaactttacaagattaaaaatcagagcaaatgaatttcttaagttcaagatatgtactctcaatggagaatcgcttttgggcagtggttaaggcctctgatgtgctacttatcagaaaaatccacatatatacaaaactctgctaaaagttttgtatccagggaaagtcccgcatccagggaaaccctcaatcccaggcactttagggcagctggtcaccctgagaacactacccactcgttccttaatatcactagagaaaaggtaagaactttcaagggcataacctttaagggcatcagtccccaaaatatttttacatcactagctaatggctagttcctctaagcttgctaaaaggctaggaagtccagaaataccttaaacgtgttaactttaagaagagttggtagtaatcaagcaaattagtgagcagtgtataaaagctcactcttgaaatctgttttcagacaaatcttctaaaggttcttctagctttgtccagttatatggtattttactgtattctctttttgcaattaatccagttttgtatgtcttttctttcttttttaggtgaaaatattctatgccaactgttttccacagtcctgcattatatattaaaacaaaggctgccagctggagacacagccctccgattacaaaggcccagaatgttacttttaactgtgctccaccaggaggtctggccttgggaaaagatggcgaaaggaatattctcagatatgaacattttttattctgcctacaatgctgtgatctagttcaacaactgcagaactgttctcatcttaatcgctgtagtttttctttctttactcttttgtataaaaggttagtgtcacagcttcactatcactaataaaaagatacaaatatgcctttcaagtcagggttggaaaagcaaaactgaggtgtgaggttacactggtctaagaaagtaccaatttgggttctatattttgtcaaacagttgggtttttaaaaaaattcaaaactcatgcatgttacctacttgtcatgtgtgaattatttctcacaattttaattaatctgtgtgtatattagttatataaagcaatggatttccacattcttaaagcaggaacctatattcaccagaaaaggatcctcctgtttctcatcaaattttttttcagctcgaacaatccaagattgggaatagtaagagtggcaaacaaatgttttcttagggacttactgagaaaagaaaaaacttactgggagaacagagacttagtaaaatttctattgctacagacaaatgctaaaaaccagctttataataacagcattataaaggatagaacttaatatagaaccagaaatatggcaagttacctagtgattaacattgtaaaatagtcaaaaactttaaagccacagagaaaggaaaacaattatgaaatggaaaatatataatatttaagtacttttataattctaaaacttcacttttgtccttaaatcaatatattacggatttcattgttcaataaattaccatctttaattaaaaataagtaaatcaaagagcatatttggagaaactaagagctgttaactgtttggagggtaaaagaatacttttctcgaaatttttttgaagaaaaatctaaaagccctctatgttgagttaatacaccttctgacccccatcatcagtggcattattcttccaagggactcttatatctaagcaatggtgaagttctggattcattatggatctcatggcaccaaaccaactggcactgaagttaagttaatatactccagcgagatcacctgtgggtcaaggatggcccagagaatcttggaaaatccatttatattgagcaaagatctgaatcaccttcaatcaggctgtaagatactagaaaatttgaccttgtagtagtatttcccagggtaacttaagcagcaaccttgcaccagaagaagaattaaagagggagcaatctagtattatcaacaacaacaaagttaaccctaagttagtacatcccagaatctgctggatgtataataatttagtaacggggtatatggcagagctttctttgatgttaacaaattttggctgtgattcttagttaccaagttgccaaaaaatggtatattaaatgaactgccaaatggcagattaagaaaattaatgtactccaatggtctgtccatgaaaggaaaatgtacacagacaaattaagaacattttaccaggatctgagatttaaacaatggaacaattgttttaactgttagaatgaccccaactgttaagtttgtctatgagtgtatatgtatatataaattcatacacatatattatttatttccttcttaaaaagactgaggcagttctgctatatatagttagctacaatattcaagataaaacagttcctactcaaaaaattacatgaacacacgagataagttcttatcgtaaatgctatcatgaggctatctagtatagctcatatttcctggttgtaaggctcaaaacacaggaattccactccaagagataatttgcccctcaatccctacaaagtgtagtctaaacaaacaaaatggtaataaaaaattgaaaaggaagatataaaaagaactcaatagcaggattctgactacctctggagaccacacactatcattattctgactgtcttaaatacaacaatccaatatgccccaagatggaaatctggtatcgtagggaaaacattggctgcaactgtcagaaaagttcataatcttaaacataatttatgccatttgccagtcacaaagacatttactgaacagaatttttgagccatttgtaaaattaaaatgattgatcaatttgaatagcaaccttcatgatgaagaaattaggactctaggtatgaaaagcatgttccttttttgttaataagttcaaaggagagaaacattctgatatatgcagataaaaatatggctaggctgggcgcggtggctcatgcctgtaatcccagcactttgggaagccgaggtggacagatcacgaggtcaggagatcgagaccatcctggccaacacggtgaaaccccgtctctactaaaaatacaaaaaattagccgagtgtggtggtgggcgcctgtagtcccagctacttgggaggctgaggcagaagcatggcgtgaacccgggaggcggagcttgcagtgaaccaagatcgcaccactgcactccaggttgggcaacagagcgagactccctctcaaaaaaaaaaaaaaaaaacaaaaaacaaggctaacaagaaagaggataaccagcaagtaccacctggatgtgtgttgtcaggtagaaaggaagaataaaattcaggcaatgaatataatagatttagcaaagtaaagcatatgaaaggaagaaatgtttgatatgtctaagtatcaatgccttcgatcagagtaagaaaaaagtattcattgttcatgtccacagactagatatctaaagagatacttggtgggcaggggcttgggagggaaggcgcaaattggaatgttcagcttttaaagtaaagactgtacatgaagacatattttatgtacagtgaagattgtcttgtgttactttatatcccaacataaacctacgccaccctcagacgaagagggtatctaacactgaataaatgctgaacctatttagtagttaaagaaaaaagagaaggatcttaaaggtatatatgggaagcttttaagaggtagagaaaccaactgggtatatattttcttttatttgatttcaactagcaagagactaagactgatgtttgtttgtttgttttaccttcaaagtcttagtcttaaattgacaagggcacaaaaaaagtgaaattaaaataattttaacaaaagggaaagcatttgacagtgtttaaaagacagacaaatcaagcaaaactcaatgtggcttaaggtaaaaaatacaactaggtattaaacaatttgtaaaaacttacaaagaaaatttagctttcaagaaaaattaggcagatttccttctgccaaagtgacaggtcctgaggaaaaaaaacacaacctctacaagaccaagcacagctcaagggtcagggccccgtcctagtcatctttttattattcaatatccatcacagtggctgggcaaacaacaggcatcaataaatgtttactaactgaatgtgtattataaggtataatcggtataactgatatagctcaaatctaatcatgaaagcttctttaaagtaggataaaaagagcacaatcagcggtattccagaaggtaggcctaaatccagttatatttttctaatcgttgaccagtggttataaagactttctgagcttctttttaaagcaatgaaactctttccaaaagaaaccccatgcagttcttcagtacagaataaatatgccactaagtcagtgagaactccaacagcctcccctaagccagcccccaaggtgtctctgtggaacctactggaaaaaatattactcatcttagaaatgtgatagaaagcatggccattcggttctcaggtcatcattcctagaaaattaacagtattgtgaagaataaatcctaagtaatgttgctaatttaaataaagacaaaaattcaacaaagaggggattctatcacttagaaaaatgaaaaccacacctataaatggggggaggggcagaaaacaaaaaaaaaatcaggccacagtagataaaatacaaaaaacatcatctcgttaaaaagcatcaaacacattcacacaaatgtaattacaaccaggaagtaaactgctcaacaggtataactgctcaataggtgttttcaaagagttgagtcccaatttcatactgtacagaaaaatcgcatcagaactgtagagatgcgctccactactgaaacagcatagtaggcactgcttgacctaacacagtaatgcaagagtaaccaccaagatcaggaccttctaccactttcagagttgttttctgcccctacaactgttccctaacaccattacaagttctcaagtaagaaaaagaagggcagaggctccactgagtatctcctacaggcctgatagtggtattacctaggacatttactctgctcacaagatgggtagtggaagacataattactggacagcacaaagtctggaagcaagcagcagggcactaaaacagtgagagcttacacaacaaaagcttgttaaattaagtagtactgatgtggtgcaaatgaaatttttacagcaaaggttgaggaaggagatatgttagtgagaatcacatgaagcagactatcacaaaataaggccaccttcaaaatgttatgaactgtagaaccattctgatcttcaagtttggatttgtatagaggtttctgtataaagcattaatacctaatcaggagtttcctttagtgtgaacctttttgcatttgatgctattctctttgccaggaatgcttatctcccctggctcctcacttggcttgcttctttaatgtcaggtgttagctcatgcatcctttccttagaggctttccttgatgtcctacctgaagcatcccatctgttattctccagtacagtaccctgtttatctccttcatagacaagtaagataattaagggttagtgtaactgctgtctcagcaaaggcaggaactgtagttgtcttgttcacctttacccaaagactaagaaaagttcctggtacaaacaggtgaacaataaatatttgttgaatgaataaaaaattactataccaaatttacatgaacacatacatatacacacaaatataggaaaatggggagtacccaatagaaaaccaccaaatgttgaaagtattgaaaatgatacctatagagacaggtggatatgatttcaaagaacaagtaccaaagacagcttcaaaaatatgaaaatttatgaaaagacgaccaggagtggttattttccatttctactaagatgcaaacaagaagaaatgtttaaactgcaatgagtcaacatcagacataataattatttgctgcagaatgaactagcaacagagtttcggaaatctcctctcactacagagcatgaaatattgtcaatcacaaaaccaggatcagttaagaacagctcagactgcaggtaacttataagctaaaaaacttgctaaataaatggcttttcccccaatttttaaaattctgaattcataattatgtgtagaataacaatcaatttataaactgaatacaacatactttaaaaacagatggcccatatctgctgatcctacctcagcatcacttttctaggtattttgcagaaacaattacatttacaaaaggcccatttcataatgcaatctggttactaaaccaaatcaaactactcgaagagcagaaggtctgctgttgaaatattgtaaaatacctttggaaaaacggtatttatagattagcttttttaaaaagggataaatatgtggaagtaattctagcatatccctgaaaataattatactgccacctatgcattttttatgaggtggaaggataaatcaacagactgctagattatacaagccaattattcctgttgaaatttgggcataagacaaagggactttctccatatgaattcttactgtatcccagaattaactggtgccagcagtatcaatgcaactattactggtgatgatgtcatgttatgctgttttgattatgaggacaaaaatgggaatggaaaaaagaggcttggaaaggttttcagtatggtttccttataataagatttagcagttaaaaaaaaaaacaaaaaaaaacaaaaaaccacaaaaagaatgactgtttaagccccactgaacacattaaggtcaaggatttcaaaagttaatccacttttcttcccccaagagtttatttttggtaaaaggcagaaaaattagtttttctacaggaaaatctgcttctaaataatttgaaaatcttgatatatattatatattaaaaaagacacacaaaaataacagagaagtgggaataacagattaggtactgcaactttataaaggtttgcctagatcaagaagcagcgcacacacacacctcatctatgcaaactaaaaatgtatataaacagcacaatactgtgatactggatcatgatacattacctgtacacataactactactgttattaataaacctttgggacactcagttttatgcccaataagacatcattaagtctttaaaatcttctcttcctctttaatgggagagtatttctagacactaattttcccatctaatattcaaatataggaaacagattccacaaggtgctttaattgatgagacctcaagtgctgttttctctcttgaacttttggatagtaaacagtccatagggaccacacacaatgctatgacagaagagttgttacattaagtcttttcatgggacttgattggtgaagctttatgacatgcttgagcaacgcactgaaggggatcccatctgagttaatactttgtccaaccactgtagaggtccattcagatgaagttcaatccagcaaggagtacttgttaccgtctgccttcggtattctgctccccaccctttcacaaaactcattcttatggtgcacattctagttagctgatagacggcttcaaaaccctgattaacagactgagccagaagagcagcaaattcctggttgttgaagatcttcagattacagcctggtggaattttacacactgttgcagggtgccagccatatctctgattacaattggggctctgcacaaagattgcactatcacttaggcactcagcaaaaacttccccacctatgtagtataagcgcactcctcttcctatatgccttcttgtcatttctaccgtggcatttcggttaacattggagagtaaacctaagcagaacctctctgaatttgatgggtctgtaaagccatctacagtgagtgagggctgtgatgcatggaaggtttctccaaccctctgatttaattcataatatgctatcgaacaccaaaatgcaggttctgagtaagtaactggctgtaaatccaagctatgattaacaggggaaagagtagtaggagatagttctgctggagagcctgtgtccatactttgattcaactgttggtcacttgtttctccatcttcactgatatatccaggaggtggcgtttctggaatataattactctgtggctcaattcctgctgggaagttagtgttttctggaatggagtgagtatagtcatccagaggcggaagttctgttaggatctcggtgtgtcggggcactaatactggaggcaaaactggtgtctcaactctctgatagtggtaagggtttacacatacttcatcctttttaagattaaaagcatattcgcagttttcaattgccttgagttcatgatgactgtgaagatcaggccagcgccataatcggcaatatataacatgtggcaatccttttcgatgggatacctggagacgaccatcaagagacctggtttgttcagagaagctgtaaaggcctgttgtatcccactgatctatcgtatttggtgtactcagtccccaaatttcagagcaagtgcttggtatggtaacacatttagtattacagttttgagtggtgatggctttctcaagctcatctaatcgtcctgttttctttagcttcttcaccagacttttcactgctttctcacaccacttttcttcctgcccattctgctctcctccgcctgctcctccagacccaccagctgacttcttccatcccagcagtctcttcacaactggcggcgtgaatggcaagatggacgacatgttcttaccaaaggcagcaagccacgctaggaaaacagcctcttgtatcgaacctgcaaggtggcgccaggtcccgccccgtcagatccggggggtccgggaccttttgttccttcctcttccgatgggatggagggggctgggaggggaagaggggaatgggcgattggaggcggaactgaaaacactcccggccgccgtcttcccgccccgcccccaggcccgggcccggccggcggcccgggcgcgcgggagggtaggggaagagaggggaggggaggggaggagagggaaggggaggggagggagcctggccgccgcccgcggggaaggagggggtgaggacgcgcgc

SEQ ID NO: 15643 - RNA, 20312 nt, Homo sapiens
  source 1..20312: mol_type = other RNA
gctgggattacaggcatgagccactgtgcccagcctatttgtgagtactcttaaggcaatatgatttgcctaagttcaataaaaatcggctctcgttataacaggatacaattggaaacactggttgtattaccaaggctttgattaaaatgtcatatttgagaatgtgtagaatgcctggcttcaatggttctcagcattacactgaattaaaaattatcatttcctggcaggcccaggaaccttaaaactataggtaaaatctaaagtctaccttgacttagcttcttagcctcaaggaggtttttaaatctgagattactgtgaccatactactattcttgcagacaaaatctgataaagtttacaaatctgttttattctgaacatctttggtaaaaatcagggtaactttaagtttctgaagaaagctatatgtacctgttattagatcacagctctgtaccgttttgaaactcctgttatccacctgcagactggatttgctcctgaatcctcctaatttccttcaatatttggctatgactctctaagaaaaaaaactactcccatgctctgaggcctataagctaagatgtgattaatttttaaaggagcaagtctcatgctgatgtatgggtcacacaaaagttcaccataccaaccaatgccatagctagagacattcaaactgcaaaccaggacaaaaagttgatgatttcaggctgtagacatttttcctaagacatcagagcaagaattgtattacaatttgatttattcaattggttgcctgtaagcctaggttcagggctcaaaaccattatgcaaactgggattgtcacattactattaattttgtgtatttcctttttaaactttgtatctgttatttgccaaattttctgcagaaagaagtacaattcctaacagaataatgctagcccagcactttgaggggacaacaaaggactaaggaaaaaaaattggacttaataatagactccaggtggacttagcctaagtgccactcccttaaagcctccctgccctcaaaggtggctaaaagggttttaacactgacttttagttgccaatcactcctgccaatgcaggatgcaggaccagaccaataacccgggaaaggtctattctgtcaccaagggacaatcaaagcctaactacaagatgattcatcatagatactttcggaaaaacatcttcatcaagagagggaaaggtgaaagctgtcagaatcaagagtcatgtttccaaaagccctgacaaatggagccagggaagtccatgaagagagggattttacgcactacctcaaagacccagaagaaaccacgccagcttgcacaaacactattcgcaaccttacacagaaaatacttttgggacatctgcctagaagccgattgtccaaacccgaactggcagcatccttgttattaatccttgtagccaagaataattatttcaagacaattatataatctttatctgtcctttaaaaacctgtcttcctttaccttcctgaatacacacagtttactatggcatgcatattgccttcacaatgccctattcccaaataaacatcattttcttttagaaagcctctgttatttaggttgacagttattacacctgaaaactaaattctagctgatcaataaaattctttggttctactgtatacttttatttggggatatctgcttccaaacacactaaagtacagtatactcaattttaaatatagacagtatatttaaaaaaaacataaaaagtatgtcgaacatttttaatttcaaacaccaaacttaaatagactaataacacagatcttctgtggtccacaaatcatggcaaaaaactttgttttcatatgcccattatggcttgctgactggcttactgcattttagattttccttatgattttagtagctttctctaatggaatgtgctgtgagtgaagcttcaaacattttccattgaatatacacagacatacaaataaagactggaaaaaatatacaccagtcgttttctctggttgttggaatctgggtgattttttaaagtcccatccactgggctgccagtaaaagaccacaaaatatttttgtgtatttacaggaacgtgataatcaaaagttgttgtgggaccattcaagatgagcgtggggaagggaagcccatttaaacatatattcaaggaaaaatatattaagttacctgaacatttgggtagaaatactgagcactgctatggtctgtctcccaaactgtccctcaaatgtatgatgagattttatcttcattgtggtggtgttgagagctggggcctagtgggagatgtttggttcactgaggcagatgcttcatgaatggcttggtgctgctcttgcaatgagttctcactctctcaagactagattagtccccaggagtgggttgttaaaaagagacttgtttggttgttgtgaacaagtgggttgtttgcacgtctgcttcccctctgaccttctccatcaagctatgaagcagcagcaaagcccttgccaaaagccagggccatgcccttgaacttcccagcctgtagaactgtgagcatccttcataagtgaccctgcctcagctatcctgttatagtaacacaaaacagactaagacaggcacacaaaagctgaggactgctgtcgactccactttcaagggctaccaagcacagccacatcaccaaagagaacaattcctgacctccttggaagcagaaacttgactctccgggcaagataactgttgtctttttaaaatttcagtgtcaaagttaaaacatgccttgatcagtcaaccaaattactgctaaaccagtattgggaagcttcctaaagcactccaagctcctaaaaacaggcagcatgaagtaaagcagatagcatctttgcatttaagaagtcccagaaaggttttggaaatggcattaatgtaaatgttcacattaagagaaaacggtttccctgaattgagtgattctttctactttctagtgctgtacaggataggctcagcgtttggagagtgttaacttccagtcatgtgataatggccaggagcaaccacaatgattaacctttagatagaaaacacaatcctttgcttttgtcttccttatgtatattagattaggcttctactcaatgctctgtaagttaaaacatttcaaaccaaataggccactctattaagtcccagcttgagcattcttcagcttctccacattttccattgtttgctggcaaaccagtacagtaacctgttaaatacaaagcaagggtgtggtagattgactgcatttaaggctccaattcttcacccctcctatgttctctcccttggtctaataactctgtagtgcctttccacactgggtttagccatgtggcttgtttctggtgaatgctagttagcatgaagcatgcagacatgaaagggagttatgggattgggcttggctgttgttgccttctacaacctccacaaaaacatgcttgtttaatggaggataggaggcatgtggaaaaatgccaagtccttccaggtgaggccaactccctcatgaacgaggaaagactacaactgctccagagacatctagccgaaatcacttatctaattcataaactgtttattgctgcacaccactgggtttttgtggttgctacgagttacttttgcggcaataattgctccaatatgttctatgtgacatttctgagtttaacatcacatttacaaactttcttagagaaagatttgttattagcaaagaccttcagagtaacctttgcctggtattctagactgtgcagatttagccatctaatactgagtacccacttcaggctgaatgatctctcaagtgctctcatttagttctcataaccaccctaaaaactaacttcctcattttagggaactggaggaaatgaagaactttaaggtagactgatgaaaagatttatctaaagtcacataaattggcacaatcagggtccaaaccccaggcctccgattctgagtcaaactgcattttccattacatcggaaatgaccaaggattaaaattagcagaatgttattctgtccagccattaaaatccaaaaaaaaaatttgttcaaagtaggcaattgagttttcattctattatccaaggtaactgaagtatttgactgtacaggactgcttccttcaagtgttccatccttagcattcttgttaaaaatggcctttaagatattgctattcccagtcaagaaatacccagacaactaaagagactaaaatcatgtaaatcatccatttcccagttgaatcttaaaaaaaaatttatgctcaatacctctctccagccaatcactatgtaaattgtgaattaagacattattacttggtggcaataacggttagaaaaaaagcacatccctctccctctcccgtctccccccgtctcccactttctacggtctcccactttccaccgtctccctctgatgccgagccaaggctggactgtactgccgccatctcggctcactgcaacctccctgcctgattctcctgcctcagcctgccgagtgcctgggattgcagacgcgcgccgccacgcctgactggtttttgtattttttggtggagacggggtttcgccgtgttggccaggctggtctccagctcctgaccgcgcatgatctgcccgcctgggcctcccgaggtgctgggattgcagatggagtctcgctcactcagtgctcaatgttgcccaggctggagtgcagtggcacgatctcggctcgctacaacctccacctcccagccgcctgccttggcctcccaaagtgcggagattgcagcctctgcccggccgccaccccgtctgggaagtgaggagcatctctgcctggctgcccatcgtctgggatgtgaggagcccctcagcccggccgcccagtctgggaagtgaggagcgcctcttcccggccgcccatcgtctgagatgtggggagcgcctctgccccgccgccccgtctgggatgtgaggagtgtctctgcccgaccgccaccccgtctgggaggtgaggagcgtctctgcccggccgccccgtctgagaagtgaggagcccctccgcccagcaaccaccccgtccgggaagtaaggagcgtctccgcccagcagccgccccgtctgggagggaggtggggggcagcccctgctcggccagccgccccgtccgggaggtggggggcaacccccgcccggccagctgccccgttcgggaggtggggggcagcccccggccagcatccaccccgtccgggaggtgggggggcgcctctgcccagccgccccgtctgggaagtgaggagcccctctgcccggccgccaccctgtctgggaggtgtacccaacagctcattgagagcgggccatgatgacgatggcggttttgtcgaatagaaaagggggaaatgtggggaaaggaaagagagatcagattgttgctgtgtctgtgtagaaagaagtagacataggagactccattttgttctgtactaggaaaaattcttctgccttgggatgctgttaatctataaccttacccccaaccccgtgctctctgaaacatgtgctgtgtccactcagggttaaatggattaagggcggtgcaagatgtgctttgttaaacagatgcttgaaggcagcatgctcgttaagagtcatcaccactccttaatctcaagtacccagggacacaaacactgcagaaggccgcagggtcctctgcctaggaaaaccagagacccttgttcacatgtttatctgctgaccttccctccactattgtcctatgaccctgccacatccccctctccgagaaacacccaagaatgatcaataaatactaaaaaaaaaaaaaaaaaaaaaaaaaaagactttagttcaagttgagaccaaagactgtgctattatggggtggagaaaagtatcacaattttggtaatactaggcaagatgtaacctcaagtctccaggcagccccatgagcttccctgtgaatgagaacagaaaaagttcaggagccaccagaggatgttaaggaggcttcctagagaagacgtggcaatgcacctgatggagacgtttaatttcttcactacaaggaatttcaaacttatctaaaaggaaatagaatacaacaaagctcccttacccaatcccaacaaacaaccatcaatgtcctattcattcatacctccatctacttcctctgtcacatactattttgaagcaagtcttacccattgtattttacccataaatgtttcattctgtatctctaaaacattgtctctagacctcagcaaaaaaaaaaaagcacatccacttttacaatggtcacatacaaatggggaaagagtggatataaaaaatatgcacccaccttcaatcaaatgcgatcttttaaagaatataaacaagccagattcttaggtatctctcccttttgtaattttgattctgaaaaaatatttaaagtaatcaattaggtattctaaaagaaggcagttttctaggggtttatttaattataggggggttggggtagagagattaaaaacgggaagcagtgcataggcagtatgaagtagacactttggcaaataaaaactgcaccgtatgacatgtcacatagaaattgttagagactttgaatcctaaaatttagtttaccaaatgtagctttttatgttttatgttttaccaacaaataatttgtatgttaaatttaagcatctgaattccgaaatgataaagaacaggaaaataatgactaagctaacaaccaaactttcagagtataaaattttgtcagtggttttcattttagaattaaaaatttgaatttccctttgcctacaagtctaagtaacttgcagcagcaaattcccccactgacaacttcaaagcatagcaagaatccacagtggtttgcaggccactaattcttttacagatgaaagcattcaattatctctataaaattcaattccttagaatatgtgtttgtgattgacgatgtacatttttaaatgtggtgataacacgttattattcatgatttaaaagttgaaatgaagtagcttgtggttcttgggtaaaacagacactaataagttttttttcaatataaaagagcaacctagacattcctataaaacatttttattccaggtggtaagctggcttaaattttcacttttcagccaggcatgatggctcacgcctgtaattccagcactttgggaggccgaggcaggcaaatcatctgaggtcaggagttcaagaccagcctggcaaacatggtgaaaccctgtctccactaaaaatacaaaaagtagttgggcgtggtggtgtgtgcctgtaatcccagctactcaggaggctaaggcaggagaatcacttgaacccaggaggcgaggctgcagtgagccgagatcgccccactgcaccccagcctgggcaacagagcaagactctgtctccaaaaaaaaaaaaaaaaaattcgtttttctcacagcagcacatttctaaatggcaaaccatttagaagtgagtcatcatttgtattaaaatcttatttacatggtacttatgtagtttgatcaaatactgccacaatatagtttagaggcaagacctctcatgaagaaaaactttacaagatttaaaatcagagcaaatgaatttcttaagttcaagatacgtactctcaatggagaatcgctgttgggcagtggttaaggcctctgatttgctacttattagaaaaatccacatatatacaaaactctgctaaaattccaatggcttctctagatgaatcatctttggctgtgagcaaaaaagttaactaagtttcacttaatacacacacacacactagggtttatatgtagcaacttcctcatcctcattccacaggtagcccgttcttggctgggttatggcttgtaatctcagaaccactgcccccaaatgactgctcagaagcacaatctcactgcaaactatggaacccaaactatacagctatccttggcttttaactccaagctatctaggccttgtgattatatgtgggcttcatagcagaacctaccaggcttgtggttatcaattttctgctcaccatataagcagtagctcaataacaccgtccagttttcatgtatatccagacacacaggtgagagttctgttccaagatctcattttgaccttcttcaaaggtcttctccatctctccaaattgaatgtattcttcaaccctgggcttactgtattctgcccatcttcttcctggaccaaactgttcagaagttaacttctttttcctgtcatcacatctctttcctaaactactttagaacttaaataattttattttcacataacatttagaaaggtgcagaggcagccaacaaaactattgaagacagactgtaaaaactggcaaatccccatctcaaattccatttattctataaccaataaagtcatgcagtttggacgggagcacagtaatacattctgttctcatgtagcttcctaagtatgcttagtctattgttcatttatcactgaatctgttatctgctaagtctgattcaatgttcttgccttctattaatgtgattttaagaattactgcatgtctcactatggcaaaatagcatgacatttgttttacaaaatcagttaaaccaattctacaaatatttccatacctatttattgcagcaaaagataatttttatgtgtaaattagctttttgggtttttctattcctttatttgtaaacttataatttttaggttgggcttactattttgatgagaagggtgaatctgtcaaagggtaagctggataactgtatgttgcaaacatgttcctgaacattcttcacccaaacttagacaaacctggagcttaaaataattacattggatgacatcagtttgatactgatgcctgcttcctgcactaagaggctttcaatctattttgaagagggaaaaacagaatatgccaagtggggagacagcccaaacatagaccttaatacttctctcatactcttcagccatttgatgaacatgtggaattatggatgctagggccattataaaaatctcctgatacagaacagtgtcactacttcaagctaagcagtgacaggcaaagccaggctgaggtgacaatgtagaaggatctcgagtcagccctcaatgttgttgttcaatgttgggaagtcccttttagattatttatacagtggcaggtggtagcaattacagtaaattttcttgggtttcttcctaataaaaaagtgttgataaaactacaccagtcccaaggctattcaatgccacgtaaaatagtgtattttagcatttgaggtccctttttgttgcatactaaagcatgtttaaaatggtttgcagaaaacagtctgctaaccagtactgattcatccacagaactgaattcttgcaaggcacaaaggaagtgtggctgacctaaatatttctcatttttaaaattattcatactgattatatgagattatatcttatctagtatttttcaatggagccttaaaaatgttattttgttaaaagtatatttcagcaaatttcaactttgaagatgtttttgtttacagcatagatcttatgtattagagcgctaatgtagcataggcaaactctgaaataaataaaaatgtataaatagcactgtgcagtgtgtggtgtgcgcctgttgtggggttatattaagtagtataaatttatctcccggggggataggataatcttttatgtaacaccaaattaaaaaaacaaaaacatgtactcttaaaatcatatgtccatatgtgaaatacaatcactttttttggtttccatataatttagggagtgaacaccaaaatgtaatcccatataaaaaaagatcagtttaaataaaaattaaaacaattaaaaattagtcccatagtaacatggtaaacaactcaaatggctttcttttaatgctaggaaaactgtccacctttcaacggtgacagggctgttaacacaggtaagagcaaacaaggtaaaaagtgaaagcacatacagatgatgcacacaaatatatataaaaattgaccagaaatcacaggacatgtaagcaatgttttcttaagcagaactttttttgtactttaaatagactaaaatatttggtgtaggtgggagaaagacatcagtattcaacaattttaacttgaaaaccagctgtaataaagcctcagctcattgtttaataaaaataaaaaaggaaccacatcgtacttttgacaatcatagaacgaaagctcacaaagaacacatttaatatctccatcacagtgcaccaaggatgcagccactaaggacttccagagggaaacaagaacagggtctgcatccatcatattgcattacaaagttaatgccatcagagaaaaaaaatctcacctcacgtgctcaatgttctagctggtaagcaccttatgagtatgaggctacaattgagagaaactgctcagtctgcatcaggacacccaattccttcacttgccattggctgatgcatttaatcattttaacacaacattcacggaaaaatgttaacaacacattctggcttctcgagcagaacagactgggaaatgcagtagacgccagagcatcaaaggccatgtatttcctcacaagaaaagaaatctgcaacaattggtttccttttactatgaaaaatgtaaatttcagattaagtttaaccccataaggacgcatgatttgtacttacatatacacataggttcagaagaacttagctatctagttggcctcttctctgttccattataacatcagttaccttagctggatcactaagtgtgagtctcaccaccatactggtaccttcagctattacctgtgttataaatctcatgttccattcaaagtactaaatgactggatggcacatatcccaataagtatcagaaatgttgacagccatagtgcagctgagtttagaagcaactatgacaacatagggaagtaaggataaatcacaagaacacctaaggtggtcagctccttctggtgtgcctgggacttgttttgagtttagcaaaaactttacaagattaaaaatcagagcaaatgaatttcttaagttcaagatatgtactctcaatggagaatcgcttttgggcagtggttaaggcctctgatgtgctacttatcagaaaaatccacatatatacaaaactctgctaaaagttttgtatccagggaaagtcccgcatccagggaaaccctcaatcccaggcactttagggcagctggtcaccctgagaacactacccactcgttccttaatatcactagagaaaaggtaagaactttcaagggcataacctttaagggcatcagtccccaaaatatttttacatcactagctaatggctagttcctctaagcttgctaaaaggctaggaagtccagaaataccttaaacgtgttaactttaagaagagttggtagtaatcaagcaaattagtgagcagtgtataaaagctcactcttgaaatctgttttcagacaaatcttctaaaggttcttctagctttgtccagttatatggtattttactgtattctctttttgcaattaatccagttttgtatgtcttttctttcttttttaggtgaaaatattctatgccaactgttttccacagtcctgcattatatattaaaacaaaggctgccagctggagacacagccctccgattacaaaggcccagaatgttacttttaactgtgctccaccaggaggtctggccttgggaaaagatggcgaaaggaatattctcagatatgaacattttttattctgcctacaatgctgtgatctagttcaacaactgcagaactgttctcatcttaatcgctgtagtttttctttctttactcttttgtataaaaggttagtgtcacagcttcactatcactaataaaaagatacaaatatgcctttcaagtcagggttggaaaagcaaaactgaggtgtgaggttacactggtctaagaaagtaccaatttgggttctatattttgtcaaacagttgggtttttaaaaaaattcaaaactcatgcatgttacctacttgtcatgtgtgaattatttctcacaattttaattaatctgtgtgtatattagttatataaagcaatggatttccacattcttaaagcaggaacctatattcaccagaaaaggatcctcctgtttctcatcaaattttttttcagctcgaacaatccaagattgggaatagtaagagtggcaaacaaatgttttcttagggacttactgagaaaagaaaaaacttactgggagaacagagacttagtaaaatttctattgctacagacaaatgctaaaaaccagctttataataacagcattataaaggatagaacttaatatagaaccagaaatatggcaagttacctagtgattaacattgtaaaatagtcaaaaactttaaagccacagagaaaggaaaacaattatgaaatggaaaatatataatatttaagtacttttataattctaaaacttcacttttgtccttaaatcaatatattacggatttcattgttcaataaattaccatctttaattaaaaataagtaaatcaaagagcatatttggagaaactaagagctgttaactgtttggagggtaaaagaatacttttctcgaaatttttttgaagaaaaatctaaaagccctctatgttgagttaatacaccttctgacccccatcatcagtggcattattcttccaagggactcttatatctaagcaatggtgaagttctggattcattatggatctcatggcaccaaaccaactggcactgaagttaagttaatatactccagcgagatcacctgtgggtcaaggatggcccagagaatcttggaaaatccatttatattgagcaaagatctgaatcaccttcaatcaggctgtaagatactagaaaatttgaccttgtagtagtatttcccagggtaacttaagcagcaaccttgcaccagaagaagaattaaagagggagcaatctagtattatcaacaacaacaaagttaaccctaagttagtacatcccagaatctgctggatgtataataatttagtaacggggtatatggcagagctttctttgatgttaacaaattttggctgtgattcttagttaccaagttgccaaaaaatggtatattaaatgaactgccaaatggcagattaagaaaattaatgtactccaatggtctgtccatgaaaggaaaatgtacacagacaaattaagaacattttaccaggatctgagatttaaacaatggaacaattgttttaactgttagaatgaccccaactgttaagtttgtctatgagtgtatatgtatatataaattcatacacatatattatttatttccttcttaaaaagactgaggcagttctgctatatatagttagctacaatattcaagataaaacagttcctactcaaaaaattacatgaacacacgagataagttcttatcgtaaatgctatcatgaggctatctagtatagctcatatttcctggttgtaaggctcaaaacacaggaattccactccaagagataatttgcccctcaatccctacaaagtgtagtctaaacaaacaaaatggtaataaaaaattgaaaaggaagatataaaaagaactcaatagcaggattctgactacctctggagaccacacactatcattattctgactgtcttaaatacaacaatccaatatgccccaagatggaaatctggtatcgtagggaaaacattggctgcaactgtcagaaaagttcataatcttaaacataatttatgccatttgccagtcacaaagacatttactgaacagaatttttgagccatttgtaaaattaaaatgattgatcaatttgaatagcaaccttcatgatgaagaaattaggactctaggtatgaaaagcatgttccttttttgttaataagttcaaaggagagaaacattctgatatatgcagataaaaatatggctaggctgggcgcggtggctcatgcctgtaatcccagcactttgggaagccgaggtggacagatcacgaggtcaggagatcgagaccatcctggccaacacggtgaaaccccgtctctactaaaaatacaaaaaattagccgagtgtggtggtgggcgcctgtagtcccagctacttgggaggctgaggcagaagcatggcgtgaacccgggaggcggagcttgcagtgaaccaagatcgcaccactgcactccaggttgggcaacagagcgagactccctctcaaaaaaaaaaaaaaaaaacaaaaaacaaggctaacaagaaagaggataaccagcaagtaccacctggatgtgtgttgtcaggtagaaaggaagaataaaattcaggcaatgaatataatagatttagcaaagtaaagcatatgaaaggaagaaatgtttgatatgtctaagtatcaatgccttcgatcagagtaagaaaaaagtattcattgttcatgtccacagactagatatctaaagagatacttggtgggcaggggcttgggagggaaggcgcaaattggaatgttcagcttttaaagtaaagactgtacatgaagacatattttatgtacagtgaagattgtcttgtgttactttatatcccaacataaacctacgccaccctcagacgaagagggtatctaacactgaataaatgctgaacctatttagtagttaaagaaaaaagagaaggatcttaaaggtatatatgggaagcttttaagaggtagagaaaccaactgggtatatattttcttttatttgatttcaactagcaagagactaagactgatgtttgtttgtttgttttaccttcaaagtcttagtcttaaattgacaagggcacaaaaaaagtgaaattaaaataattttaacaaaagggaaagcatttgacagtgtttaaaagacagacaaatcaagcaaaactcaatgtggcttaaggtaaaaaatacaactaggtattaaacaatttgtaaaaacttacaaagaaaatttagctttcaagaaaaattaggcagatttccttctgccaaagtgacaggtcctgaggaaaaaaaacacaacctctacaagaccaagcacagctcaagggtcagggccccgtcctagtcatctttttattattcaatatccatcacagtggctgggcaaacaacaggcatcaataaatgtttactaactgaatgtgtattataaggtataatcggtataactgatatagctcaaatctaatcatgaaagcttctttaaagtaggataaaaagagcacaatcagcggtattccagaaggtaggcctaaatccagttatatttttctaatcgttgaccagtggttataaagactttctgagcttctttttaaagcaatgaaactctttccaaaagaaaccccatgcagttcttcagtacagaataaatatgccactaagtcagtgagaactccaacagcctcccctaagccagcccccaaggtgtctctgtggaacctactggaaaaaatattactcatcttagaaatgtgatagaaagcatggccattcggttctcaggtcatcattcctagaaaattaacagtattgtgaagaataaatcctaagtaatgttgctaatttaaataaagacaaaaattcaacaaagaggggattctatcacttagaaaaatgaaaaccacacctataaatggggggaggggcagaaaacaaaaaaaaaatcaggccacagtagataaaatacaaaaaacatcatctcgttaaaaagcatcaaacacattcacacaaatgtaattacaaccaggaagtaaactgctcaacaggtataactgctcaataggtgttttcaaagagttgagtcccaatttcatactgtacagaaaaatcgcatcagaactgtagagatgcgctccactactgaaacagcatagtaggcactgcttgacctaacacagtaatgcaagagtaaccaccaagatcaggaccttctaccactttcagagttgttttctgcccctacaactgttccctaacaccattacaagttctcaagtaagaaaaagaagggcagaggctccactgagtatctcctacaggcctgatagtggtattacctaggacatttactctgctcacaagatgggtagtggaagacataattactggacagcacaaagtctggaagcaagcagcagggcactaaaacagtgagagcttacacaacaaaagcttgttaaattaagtagtactgatgtggtgcaaatgaaatttttacagcaaaggttgaggaaggagatatgttagtgagaatcacatgaagcagactatcacaaaataaggccaccttcaaaatgttatgaactgtagaaccattctgatcttcaagtttggatttgtatagaggtttctgtataaagcattaatacctaatcaggagtttcctttagtgtgaacctttttgcatttgatgctattctctttgccaggaatgcttatctcccctggctcctcacttggcttgcttctttaatgtcaggtgttagctcatgcatcctttccttagaggctttccttgatgtcctacctgaagcatcccatctgttattctccagtacagtaccctgtttatctccttcatagacaagtaagataattaagggttagtgtaactgctgtctcagcaaaggcaggaactgtagttgtcttgttcacctttacccaaagactaagaaaagttcctggtacaaacaggtgaacaataaatatttgttgaatgaataaaaaattactataccaaatttacatgaacacatacatatacacacaaatataggaaaatggggagtacccaatagaaaaccaccaaatgttgaaagtattgaaaatgatacctatagagacaggtggatatgatttcaaagaacaagtaccaaagacagcttcaaaaatatgaaaatttatgaaaagacgaccaggagtggttattttccatttctactaagatgcaaacaagaagaaatgtttaaactgcaatgagtcaacatcagacataataattatttgctgcagaatgaactagcaacagagtttcggaaatctcctctcactacagagcatgaaatattgtcaatcacaaaaccaggatcagttaagaacagctcagactgcaggtaacttataagctaaaaaacttgctaaataaatggcttttcccccaatttttaaaattctgaattcataattatgtgtagaataacaatcaatttataaactgaatacaacatactttaaaaacagatggcccatatctgctgatcctacctcagcatcacttttctaggtattttgcagaaacaattacatttacaaaaggcccatttcataatgcaatctggttactaaaccaaatcaaactactcgaagagcagaaggtctgctgttgaaatattgtaaaatacctttggaaaaacggtatttatagattagcttttttaaaaagggataaatatgtggaagtaattctagcatatccctgaaaataattatactgccacctatgcattttttatgaggtggaaggataaatcaacagactgctagattatacaagccaattattcctgttgaaatttgggcataagacaaagggactttctccatatgaattcttactgtatcccagaattaactggtgccagcagtatcaatgcaactattactggtgatgatgtcatgttatgctgttttgattatgaggacaaaaatgggaatggaaaaaagaggcttggaaaggttttcagtatggtttccttataataagatttagcagttaaaaaaaaaaacaaaaaaaaacaaaaaaccacaaaaagaatgactgtttaagccccactgaacacattaaggtcaaggatttcaaaagttaatccacttttcttcccccaagagtttatttttggtaaaaggcagaaaaattagtttttctacaggaaaatctgcttctaaataatttgaaaatcttgatatatattatatattaaaaaagacacacaaaaataacagagaagtgggaataacagattaggtactgcaactttataaaggtttgcctagatcaagaagcagcgcacacacacacctcatctatgcaaactaaaaatgtatataaacagcacaatactgtgatactggatcatgatacattacctgtacacataactactactgttattaataaacctttgggacactcagttttatgcccaataagacatcattaagtctttaaaatcttctcttcctctttaatgggagagtatttctagacactaattttcccatctaatattcaaatataggaaacagattccacaaggtgctttaattgatgagacctcaagtgctgttttctctcttgaacttttggatagtaaacagtccatagggaccacacacaatgctatgacagaagagttgttacattaagtcttttcatgggacttgattggtgaagctttatgacatgcttgagcaacgcactgaaggggatcccatctgagttaatactttgtccaaccactgtagaggtccattcagatgaagttcaatccagcaaggagtacttgttaccgtctgccttcggtattctgctccccaccctttcacaaaactcattcttatggtgcacattctagttagctgatagacggcttcaaaaccctgattaacagactgagccagaagagcagcaaattcctggttgttgaagatcttcagattacagcctggtggaattttacacactgttgcagggtgccagccatatctctgattacaattggggctctgcacaaagattgcactatcacttaggcactcagcaaaaacttccccacctatgtagtataagcgcactcctcttcctatatgccttcttgtcatttctaccgtggcatttcggttaacattggagagtaaacctaagcagaacctctctgaatttgatgggtctgtaaagccatctacagtgagtgagggctgtgatgcatggaaggtttctccaaccctctgatttaattcataatatgctatcgaacaccaaaatgcaggttctgagtaagtaactggctgtaaatccaagctatgattaacaggggaaagagtagtaggagatagttctgctggagagcctgtgtccatactttgattcaactgttggtcacttgtttctccatcttcactgatatatccaggaggtggcgtttctggaatataattactctgtggctcaattcctgctgggaagttagtgttttctggaatggagtgagtatagtcatccagaggcggaagttctgttaggatctcggtgtgtcggggcactaatactggaggcaaaactggtgtctcaactctctgatagtggtaagggtttacacatacttcatcctttttaagattaaaagcatattcgcagttttcaattgccttgagttcatgatgactgtgaagatcaggccagcgccataatcggcaatatataacatgtggcaatccttttcgatgggatacctggagacgaccatcaagagaccttggtatggtaacacatttagtattacagttttgagtggtgatggctttctcaagctcatctaatcgtcctgttttctttagcttcttcaccagacttttcactgctttctcacaccacttttcttcctgcccattctgctctcctccgcctgctcctccagacccaccagctgacttcttccatcccagcagtctcttcacaactggcggcgtgaatggcaagatggacgacatgttcttaccaaaggcagcaagccacgctaggaaaacagcctcttgtatcgaacctcccggcggctggcgggctgctggctggcgagctgcttctccgccgccgcggccgcgcgggtagacccgcct

SEQ ID NO: 15644 - RNA, 6091 nt, Homo sapiens
  source 1..6091: mol_type = other RNA
gctgggattacaggcatgagccactgtgcccagcctgagctgttaactcttaatctaaacaatgccttttacatgagaaacagtaaacaagatggcaagggatggcaaagaggatactgaaatatgttaggagctacatacaagaaataaattcacagttaaaagatgaagacctttatctaaatccaggcaaactgcaaactttaaaaagaattatgataagaataaagcatcaggaaggagaaagacaaactgatgacactgatatcccagaataaggccccatagacaaaggtataaccatcatcacatatggttggtgactcccacagcgtgttcctcaccttccccagtgcctttgggaaatgtgagtgttctctgtaaaagttctggcatggtgaaagatcgtaactctaggaagctgaataacttaccatttggcactaatatccctgatttcttctgtttaacttttttgctctcatctcccttaatgtatcattctgttgtcacgaagtgaatgcagttgccattattcctgtattagagtgctaggcctatcttcattttgttgagttgaattttatagctgctgaagccagggttacatcttttagcaagaataaattggtggttggaatagaaaaagtatagtaacttttgttgcactgtgacaatagattttatctggcatggtaatgccaatcaacttggcatcatttcctggctcagcgagttggaataattatgagaatccattcagagtctgtggggaaaactgctaggattgattagcaatgtctaccattggaaaagtagagaattgttggcttttatgacatagacagtttgccgattctgctttagcttacatgcataacagcatacttttttttaaaccattcttttgcttagtagccataaaaatcaatttggcttatttaaaagtttcataatgaaacatacctatttacctataggtttcttttgccagatattatattaacaacttttcttaaaaataattttattttttgaaaggaactaaataatgtcagtatatagatgctgctgtactatcattaaggaagcatgtgctgaggttgtgttctcagaaacaaggaagaatgacatttgtccagtcatggagctctgtggctccatgcagggccatgaatttgttgatgtctgtgatgtacagtcatggaacagagagaagctaactgacccatgataagttaaacctcaaatcttaccacttttaatgccacagtaaaattttctaaactggtcaaccacaacaaaagtatatttaaaaactaatatgaagtatatcaagaatttaagaactgctgtttcatgaacctatggaatggcagatctgaaagtcatcgtggagatcgtttagaccaggagcttgcaaacgatagccagtgggccatatccagcccactgcttgtttttgtaaatcaagttgtactggaatactgccaggcttatttgtttatgtattatctgtggctgcttgtgcactatagtgacccagttgagtaaatgcaacaaggctatatggaccacaagcctaccacatataccgaggctatatgaaccacaatgcctaacacatttactatctggccttttattgaaaaagtttgccaactcccgattttaaccaacttttcattttagaattatggaaattagaaatcacagaggttgtgtaacttgtttgggataattctaccacttgagaaaatagccaacagaattcccagaacccccagtggcaggatccagagctgcagtctcaagagctgcagtctctatctgaaagagagcattttcacgtctctggaagccctaccctaccttgtcagccatgctgccactccctccctccccacttcacacacttaatgcaataaaggcaaaatgaatacatggatgaaaactctcctgtattcatagaatatttctcacattccttcatcattccaagtattatacggaattgtaatcatttgcctttcccactagaacatgagtgcactggggacagggacaatgccatatttgtctttgtatcccagatgcttagcacagattacagaataggtatctattacctgtttgttaaatgctttggatttgctatcttatcttcttccatgcccattttaagataaacttcaactacagggaagataaatgcaagttgtggtttgtaattttcatcattcctgaccaagacccaccactgagacccaacaataggagatatccagaaccaaacaccatgataggaaagttacaaatctgtttttttcattgcacctactaaggaatggcccaaagcctccaaggcaatcttgacctgcatccctggcaaacagatgagaacctgatgtaagtcagggataataagagtgaagaagagagagatatgaaagattattaaaatcaagaggacatcatggttgattgactgtccagggggtggttgaaagtctgtgactgcccagattctgccaagtttcagaatgcaggaggaagagcacattgggtaagggaggtgtgggtgggaagggggcatggaggtagaggcagataggatacaagcggggaggttcagtagtcaatggtatatgaagctgcagctttcatgataaacatgggttcagatgaagtcattcagagagtaaatcaagattaagagaacacaaaattaagcctagagatcaccaaaaggattgaacaaagtaaaaaggaactcccacttagaaggatcacctagagacacaggagggaggcaaaagggtagtgtcccaaaagccgtgggcagagaaaaggaaaaatgtcaagtaagatggcaaaacaatatatgcctttcatttagcaacttggtggtctgtgacaaccttcctgagagccgttttagtggaggagttgtcttggaagcctgattcaatgggtagaagagtaagtgtgaacttgggaagagacattgagtatattttactcttaagaaacttaatcgataggaagaaagagaaatgagatggtaactggaagataggtttgtattccactgagtgggtagcatcattgatttgtgaattctttgaagagaatctaccaggtgtcagaatcatagagggaaggtatataaaagccaggtgggaaaggaaacatcaccaagaagaggaggaatttatctctatgaggctaggtcttttcacttataaatggaaataataatagcttcctcagagagaagttggaggtttaaacgaaataacataatttaaaacattttgaaaacagcaaagcactattcaaaaccagattattctatatattatcaactccagttgattaccttgactcaatatctgattagtctcaatcttagagtccaattatgattaactttgtcattgcagctcagaagtcagggatcaatttccttttcctgacagtgggatatattctgatgccttggatgccagataattcttatttacttcagttatcaaattaagtaccatgtttaaagcaaatcagtggtgctgccacagtgcacatgcatagtcaatggatgttataggagatacagatgtctctgtcagtaggctaaggggtgcaagttactagcctacatgatgatacccaggacaggtaaagatgagatgatgttggtggctagacaagatttcagtcgagtaagacttcccatctccttagaattatagtagcaaagatatcatgtggcagaaatcaccagagctagactctggtgaaacccttatgctcaattttttgtgatgtggaagttccttctaggctctggtattacgaagtaaaattaaaaagccaaaatcaaaagcttactcttgtgaatcagagtgttacaactcctggtgagagaactaggaaggagatcttgattatgggaccattttctaaggagttaaatacagattgtagcaacatagatcctagattatgaaaaatgctttactaagttttgctttttttccattacacaaattcaatttgtttgaacaagattataaaaatagtaattataccctatcagctaattatttttttagaatgaatgagttataacagaagcaagcaacacagttagcaagcatcattactgtttattttcattttttcatgtatacacttacttatttatatcctatgttcttccacaaaggagccaaagtgactgttgctatttatttcatatgttgttattcataattcattacccagaagacaccagttctcttggtagtgaaatatatgttaatttaagtatttttttgcctcaaacatctcaaatagtaaattaaaatctcttatgaaataacagaagaatatacaagttctccaagtccttcaaagaataaaaatattatttacactcctgtatctgttagggttagagattggggactttaaataaaataactaaaataacaaatgaccaccaaatcccaccgtcacggacgatgggaaactaaaatcagctttaacattttcagacaatttccaacctctcatccactcctcttttgtgtcctcaccctgctccacattttgctttactctgccctgctctaagcagatggcccttgtggtcatatgtcaagatcctaaaactatttctgacctggaacaaagttctgcctgatttgatcttagttcaggtcacatgtttttctccatctattcctatgaatgtttaagaaaacttattcacttccttattaatagaacaaaaacatttgtttttgttctattgcttgctcttacatggttagccaactacaatgaaccactcactcctggggaaatcactagaaacaaagatttaatggataaaaacaccagactagtgacaattttttctgatggaaattgtttggaagttttttttttcttaaatatgaaagtagagctgtgtgacttataattaaatgctgattatcctctgtatggacatattcacaggtagctgtgtgtatacttgtatatgcacaggaaaggtgtgaaagaatacaccttcaaagagtggccatatctaagagtggggctgggagatgagaaaggagagctttcacttcctgcttcctgtatatcctgtttgaagttttacaatgatcaaatattattgttttaattaataatgtgaagaatgaaaatatttctaacattcacaaattaaagatgatagcatggttgatttgaaattttttatactttgcacagtggtgttttcaattcagtgatttatgacacattttgggctttatcctaatgcacgaatgattgaaaataaaaagatgaaacttaccctaattatcatacatatacaattcctgttagatatgaatatcttgcctcaagatttttattaaagagttctaatttagtcctatctctgtgactaggattataaccttttaatattgttaccaagatcttatacaaattactcattgaacaagcaattcattgaacaccttgtcaacccctgggctgagcattgagggcagagatgggtagacgtgagccccttcagttgtatgagctagctttcattgcatgctttccatgccccaggactctgtgtagtgctttacatatattaactcctttcatcttcacaacactcctgtaaggtataaatattattaaacccattttactcagattaagaccctgagacagatttagaatcccagaggtctagctctgactcaaaagcccatggttttaaaccgtgacttcgtagtgccttctggatcataaagtagatgtaatatagtaggagttttacaagtaaatatttaagtatattttaacatttgtaattatttaacaattggaacaactcgaatttccaacaataggaagttgattaaatacaacggagtctacccatacaatggaagacttaagaagcatttgaaatgatgatgtagaatgtagacactgatctattaacattaaaaaactatctttggcctggtgcactggctcacgcctgtaatcccagcactttgggagg

SEQ ID NO: 15645 - RNA, 766 nt, Homo sapiens
  source 1..766: mol_type = other RNA
gctgggattacaggcatgagccactgtgcccagcctgattgtttctttatgatgagactcaggttaaatatttttggcagaatattacaaataagtcatgtttcaatgccaccttttataaatgtttcttatccttctcttttaaatgtgtgaagccaggaataataaaaagtctaataatcttattttcaaatatctagcaggtcatttattggcaagtgactcttgtcatcacgtcatgattgaggcagtaggctatttatacagatcagttgatttaagggtgatccacctgggatcttctcattcatcaatccatggaatccatggaatcctgcagtgagtttctgtttcatgttccaaacagaaatatgcttctggttattcatgctatatatatgacctcttgacaacttttgatcttttgcagccttctgagagaaattgagtggatccggagccggagatattggcctcaaggtatgagccagcaacattctgagggttctaggaatggcttctcattatgggagcacttggttaaattaaactaccacagtgctcagagttctaatacagtgagctctgcaatgtgcatgaatgcagataaattacacagggctagaagaatggacttggcacctcagacaatttcagataaatcaaaatgtgctcctcatcattccatcccatgtggcctgcgcgccaccacaccacacggccacccccgcgccaccctgaaattgaccgcagcaggctgggcgtg

SEQ ID NO: 15646 - RNA, 55 nt, Homo sapiens
  source 1..55: mol_type = other RNA
gctgggattacaggcatgagccactgtgcccagcctgtccttgtgcctttgattc

SEQ ID NO: 15647 - RNA, 612 nt, Homo sapiens
  source 1..612: mol_type = other RNA
gctgggattacaggcatgagccactgtgcccagctagaggtaattaagttttgagggtggaagcctcatgatggcattagtgcccttataagagacatgagaaagaggctctctctctaggccatatgaggacacaggaagacggtggctgtctacaaatcaagaacagggacagcaccagacaccaaatctgctggcaccttgaccttagactttccagcctctggagctgtgagaagccacccagtgtatggtatttgtgataaaagcctgagctggctgggcgcagtggctcacgcctggatccacatcagaagaataaggaaaagaatggaattccaaagaactgaaagcctcgctgttggcttcttggctgggtccctgcaggacgtaatctcttatgtcacacgctgatggcaggtccaaagcactgctctcctctgacaggctgcctgaagtggcgtccctggctgccatagtccatccgcaaccggaacgcggaagcaatggcgccatcttttttatgggaaatgtgaggttcgaaggaagtcaccggagccatccttactgcgggcagtgaagggcaatggaagccggtcgcggccatgttga

SEQ ID NO: 15648 - RNA, 5419 nt, Homo sapiens
  source 1..5419: mol_type = other RNA
gctgggattacaggcatgagccactgtgcccagctagttgcttacttcttaagtgacctaatggtgacttcagtgctcgagggcacttcctaggctatttggtggccctcagtaataaagagattgtataatcttgtatactgattagccaatttatcttcgttacagtatcatcactttcatttgatactactgcaactgaaaaaactaagcctactaacatatgctaacaaaatactacttttagtgcattaaattgtaaatcaagtctgaatttccaaaattttttaaggaaaatgtttttagaaattgatgatgtttagatggccaagatgacacccattagtggttctgactgttaaaaaaaaaaattaaagaaacaaaacagactagcattcagtttctgtggaagctttctctttcttaacctttttttcttctgctgtcattccagacacaattactaagctgcttacactactggcatgtccagatctgtctaactttccctgaatggatttcacattcctaggatgtccatgtaaactttttgacctgagagatgggaatcccaaagtttgatctggcttcacagacagtaagttttccatcccatttctgtcagtaatggttagggacaagcgagggattcgaggaattgcttcagcgacatggtgttcatcttgcatatctgcaaactgctctttatgctcagcttgcactgcagcttccgacacaatgtaaggaatatctgtgctatgagagcgcgtgatcttttgaacttggcattgccattccgtcgtcaattgctggtccgtgattgaactgtactctacatcctggttaaccccaccgaccagctttcttccccgggaatagacgaagcttctggacttcattgttttacaagcattgatcgtttcatcggggaaatagcgtgtaattttggtttcttccaggggataggaaatagtgccttctatatttgtcgtttccactgttagctgagtgttttgaacatctgatttgtcctgtccatgtatcacatctgttttatttaaacttggggaaatagtttcttcttttttagagtctgtctgtctttcatcatcttcctttgaaatcccaatatctggacctaattttgactcttcagcgttctttaagtcatctactgcaaggtgactgccatctggggttgctgatgtgcttgtgcccagtgaaaggtgaagactgttctgacattctgggactaggtgcgttttcacgtccttctcttcctttatacggaaggaacaggtttttttcctgactcctgtccctggtgacgtggagagagatgtatcctcaaataataactcttctccgttaaaatgatatcgatacaagctgtagccatcagcgctattgatgctgctttgccggagaagatacgttgcctcacattcagaagaagcccgggaccgtgcctggatcaggtcagacctgtcgattcccgcaagattttcaagagcattcaccattctgttagataattcttctagctgagcaagtcgaaggtcaacagtctgcagggaagttttcataaaagtttctctttcattgatttcttccaacctcattgacatattttcaactctttcagaagtgacccggatgcgctcgtcgctggacgactgctgctcatcctccttctcccggaagtgctcctgcacgcactgctcctcgaactcatgcagcctctttagctcctcgtcgctaaggaagagcttcaatccacgatcccgttcctcttggtccccttctctctttttcctgcagcggccgctgagacgcataatgatgatgtagatgtggcttaaaatgatcatcggtgggggcaggactggcctgtcatgaaatgtcataatcagctgatatcgctggaacttccacacctggttggatattgattttacttcaaagaaggtattgttgaacacagcaatcagcaggttcaccagcaggatgttggcgaccagtagatagcacgccatgagtgctggagtgagccaggcgccggggatacagggaggaagccgcttgccctcctcatcatataggttctcaccacaaggaggattaatttccatggcgtagaggtctatctggtctgcaaacacctctccatagatcatccagtagggcatgtagaagatgtttcgggccagtttccaagagggcttctcctctggatgcagaatggcttgacgggctactccgaaactcatgagcacgaccagcatgatgaccacaaagtacagcatgtcgatcatcatctttccaatcatcatcacgtatggccccagatacttgttgacaccaaagatgtccaggacacggatgtaccagaagatgatatccacacagtagatcacccggccatagcccatgtagggctggttctgtaggcgaagaattgctccaatcatgaatgtggaaatggccacgagatctgtgatgttccagtactcctgaagccaaactttgattttctggctgagtttgcctggttctgacatgaggatctctcgtatcttctctaacgccaggctcacgatgtaggagatgacgatccactcctggagggacggccagccatccatccgcaccaggatgacgtagttaaacagcagcaggtagcccaagtatgatattgtgtaaaaccagaacttgacaatgggcgcgttatagaattcacagatctttgttccgatgggaatacttctctgttttttgtgctcgttctcctcatccccctttcttgagccagcatctgcatttgcatccgtattttcctcttctttttctttgccatcctcattttccttggatgtttgatacgagaaatcatcatatgtgcgaaattccaaaaacaagatggtggggggtagaagaatccccatgataaccttcaggccggggttcttccgcatccgcagtcttcccatccacatatcggtcagcagcatctggctgcaggtgtgagcaatgaagtcccggtgtttggctgccacggccagtttgaggcaggtcgagttgctccagtttttcagctcgtaggtcaggagtttcatagcgatctgctcgtcatgcttataggactggtctaataactccaaagcaagctggccgaagtctttggaattgttatccaagtcctgggagatgtcatccaccagatcactctcggaggactcgtgggccatggccttgtagagcttgcaggccaccagggccttggccatgctctcttcccctcgctgccagaggaacactgccattttctggcgtttcatcagcactgcccacaccatcagctcgtggaagggatactggaaccgactcacggcagggtcgtccacatcaatgtcgatctcttcctcctttttcttctttttctttttcttccctttagctggaggctcatcatcttccattcccagaagtttaagagctttaggcctctttggtccaaacaagttgttgtaaagggtccgaaagtttttccgagtgtagttgcagcggtaggctcctcccatgaggtactccagcacgagcccgatgtctatgaggctgatgtggtaatcaggcggaaggttgctctttttcacatccctcaccagcagatgaagtgtgtttggtggacccagtcttgtgttataaagctcctccagcctcggaatggtcagaaagtgttgcatgttcactccgttttcaatcaggagcttcacaaagtcgacacgatctaagactaaagcatctagcatcgcttgctccaaagcattcacccagttcagcagctctatcttccgggggtcagtttcttcctccacttcctctttcactttccctttcttcttgcctttcccttttcctcttcctcccttggtggtggccatgggtggcttcttctccttctccgtggctttgctgtccgtcgggggtgccaggcttcccaggggcggccagtggggcccaaagacaaagatctggcttcgtgctatgtccacgcggttccaagccagtgccaagctcagctgatctggagcagatacgtttgttcctttcagcagggcagttaaaattgccatctcgatgtcctgctggccctcagaacccattctgaacacagtgacgagttctttcttcttcatgcactccattataattgcaaacagctgatgtgattgtgccttattataattaaatgttttctgaatggtaactagaagctgctccctgagggactcatttattattccgccttcttcacagtacttgtgcgcaaaggacaggatgtccgaggcacgtccgctgccatcacaaatcaccacagggatgggaggctcttcttgcaggtattccaagacgatggacaccacgttagggcccccctccaccacgagacccacgaggggcacgccctgccccagtcttgtgttgatcttctgcagggagatgtgcttttccagcagccttcgcagcttcacctcggcgccatacttgcccagggtgccattgtcagccaggatgaagtgggtgtgggagttgttgagcacagagagcttacttagagggttggacatggtctggtacactcttgttacatcctttccaaccaggtcttccttattctccacgatgccccatggagcaattcctatagcacaaacccggcctctggacttggaggagtggtctttcaaggcatcccctacgtggctgataacacctgtgctgacacccccggtgaagatccaggccccggtggtcatagcagccttgatcaggcctttcccaaagacttgtttcagcttgggctgcatctcaaagttctggaggcctccatgcacagatattaagagcttggggagttccagctgccaatctttcaccatgagatggagcagtgagtctggcttggtgtcataggatacacggatatacatggctttattggaatatccgccaccctggaattcaagaactccataggaatctgttgggtagctctgggtgtgcttggcaacagaccatttctcaggctgagtctccacctgtttgctttcctcttcatttttgctgggtgttgcacttggcagaggggggatatgctggttggtgaactggccacagcaacacctgttagagtctttcatgctaggaattacaaagatacattcccgtttgcaaaaggttttctctatccaagatttctgacccatgagttttcaaaaagttgatataaggaaatagcctcagtccagcactgcaagttactgctgagtcctcagaaatcttctagaacctgccacagcagtggaatggagagggcacagctcaggctctttcagcctcctccttggccagggcaggg

SEQ ID NO: 15649 - RNA, 5333 nt, Homo sapiens
  source 1..5333: mol_type = other RNA
gctgggattacaggcatgagccactgtgcccagctagttgcttacttcttaagtgacctaatggtgacttcagtgctcgagggcacttcctaggctatttggtggccctcagtaataaagagattgtataatcttgtatactgattagccaatttatcttcgttacagtatcatcactttcatttgatactactgcaactgaaaaaactaagcctactaacatatgctaacaaaatactacttttagtgcattaaattgtaaatcaagtctgaatttccaaaattttttaaggaaaatgtttttagaaattgatgatgtttagatggccaagatgacacccattagtggttctgactgttaaaaaaaaaaattaaagaaacaaaacagactagcattcagtttctgtggaagctttctctttcttaacctttttttcttctgctgtcattccagacacaattactaagctgcttacactactggcatgtccagatctgtctaactttccctgaatggatttcacattcctaggatgtccatgtaaactttttgacctgagagatgggaatcccaaagtttgatctggcttcacagacagtaagttttccatcccatttctgtcagtaatggttagggacaagcgagggattcgaggaattgcttcagcgacatggtgttcatcttgcatatctgcaaactgctctttatgctcagcttgcactgcagcttccgacacaatgtaaggaatatctgtgctatgagagcgcgtgatcttttgaacttggcattgccattccgtcgtcaattgctggtccgtgattgaactgtactctacatcctggttaaccccaccgaccagctttcttccccgggaatagacgaagcttctggacttcattgttttacaagcattgatcgtttcatcggggaaatagcgtgtaattttggtttcttccaggggataggaaatagtgccttctatatttgtcgtttccactgttagctgagtgttttgaacatctgatttgtcctgtccatgtatcacatctgttttatttaaacttggggaaatagtttcttcttttttagagtctgtctgtctttcatcatcttcctttgaaatcccaatatctggacctaattttgactcttcagcgttctttaagtcatctactgcaaggtgactgccatctggggttgctgatgtgcttgtgcccagtgaaaggtgaagactgttctgacattctgggactaggtgcgttttcacgtccttctcttcctttatacggaaggaacaggtttttttcctgactcctgtccctggtgacgtggagagagatgtatcctcaaataataactcttctccgttaaaatgatatcgatacaagctgtagccatcagcgctattgatgctgctttgccggagaagatacgttgcctcacattcagaagaagcccgggaccgtgcctggatcaggtcagacctgtcgattcccgcaagattttcaagagcattcaccattctgttagataattcttctagctgagcaagtcgaaggtcaacagtctgcagggaagttttcataaaagtttctctttcattgatttcttccaacctcattgacatattttcaactctttcagaagtgacccggatgcgctcgtcgctggacgactgctgctcatcctccttctcccggaagtgctcctgcacgcactgctcctcgaactcatgcagcctctttagctcctcgtcgctaaggaagagcttcaatccacgatcccgttcctcttggtccccttctctctttttcctgcagcggccgctgagacgcataatgatgatgtagatgtggcttaaaatgatcatcggtgggggcaggactggcctgtcatgaaatgtcataatcagctgatatcgctggaacttccacacctggttggatattgattttacttcaaagaaggtattgttgaacacagcaatcagcaggttcaccagcaggatgttggcgaccagtagatagcacgccatgagtgctggagtgagccaggcgccggggatacagggaggaagccgcttgccctcctcatcatataggttctcaccacaaggaggattaatttccatggcgtagaggtctatctggtctgcaaacacctctccatagatcatccagtagggcatgtagaagatgtttcgggccagtttccaagagggcttctcctctggatgcagaatggcttgacgggctactccgaaactcatgagcacgaccagcatgatgaccacaaagtacagcatgtcgatcatcatctttccaatcatcatcacgtatggccccagatacttgttgacaccaaagatgtccaggacacggatgtaccagaagatgatatccacacagtagatcacccggccatagcccatgtagggctggttctgtaggcgaagaattgctccaatcatgaatgtggaaatggccacgagatctgtgatgttccagtactcctgaagccaaactttgattttctggctgagtttgcctggttctgacatgaggatctctcgtatcttctctaacgccaggctcacgatgtaggagatgacgatccactcctggagggacggccagccatccatccgcaccaggatgacgtagttaaacagcagcaggtagcccaagtatgatattgtgtaaaaccagaacttgacaatgggcgcgttatagaattcacagatctttgttccgatgggaatacttctctgttttttgtgctcgttctcctcatccccctttcttgagccagcatctgcatttgcatccgtattttcctcttctttttctttgccatcctcattttccttggatgtttgatacgagaaatcatcatatgtgcgaaattccaaaaacaagatggtggggggtagaagaatccccatgataaccttcaggccggggttcttccgcatccgcagtcttcccatccacatatcggtcagcagcatctggctgcaggtgtgagcaatgaagtcccggtgtttggctgccacggccagtttgaggcaggtcgagttgctccagtttttcagctcgtaggtcaggagtttcatagcgatctgctcgtcatgcttataggactggtctaataactccaaagcaagctggccgaagtctttggaattgttatccaagtcctgggagatgtcatccaccagatcactctcggaggactcgtgggccatggccttgtagagcttgcaggccaccagggccttggccatgctctcttcccctcgctgccagaggaacactgccattttctggcgtttcatcagcactgcccacaccatcagctcgtggaagggatactggaaccgactcacggcagggtcgtccacatcaatgtcgatctcttcctcctttttcttctttttctttttcttccctttagctggaggctcatcatcttccattcccagaagtttaagagctttaggcctctttggtccaaacaagttgttgtaaagggtccgaaagtttttccgagtgtagttgcagcggtaggctcctcccatgaggtactccagcacgagcccgatgtctatgaggctgatgtggtaatcaggcggaaggttgctctttttcacatccctcaccagcagatgaagtgtgtttggtggacccagtcttgtgttataaagctcctccagcctcggaatggtcagaaagtgttgcatgttcactccgttttcaatcaggagcttcacaaagtcgacacgatctaagactaaagcatctagcatcgcttgctccaaagcattcacccagttcagcagctctatcttccgggggtcagtttcttcctccacttcctctttcactttccctttcttcttgcctttcccttttcctcttcctcccttggtggtggccatgggtggcttcttctccttctccgtggctttgctgtccgtcgggggtgccaggcttcccaggggcggccagtggggcccaaagacaaagatctggcttcgtgctatgtccacgcggttccaagccagtgccaagctcagctgatctggagcagatacgtttgttcctttcagcagggcagttaaaattgccatctcgatgtcctgctggccctcagaacccattctgaacacagtgacgagttctttcttcttcatgcactccattataattgcaaacagctgatgtgattgtgccttattataattaaatgttttctgaatggtaactagaagctgctccctgagggactcatttattattccgccttcttcacagtacttgtgcgcaaaggacaggatgtccgaggcacgtccgctgccatcacaaatcaccacagggatgggaggctcttcttgcaggtattccaagacgatggacaccacgttagggcccccctccaccacgagacccacgaggggcacgccctgccccagtcttgtgttgatcttctgcagggagatgtgcttttccagcagccttcgcagcttcacctcggcgccatacttgcccagggtgccattgtcagccaggatgaagtgggtgtgggagttgttgagcacagagagcttacttagagggttggacatggtctggtacactcttgttacatcctttccaaccaggtcttccttattctccacgatgccccatggagcaattcctatagcacaaacccggcctctggacttggaggagtggtctttcaaggcatcccctacgtggctgataacacctgtgctgacacccccggtgaagatccaggccccggtggtcatagcagccttgatcaggcctttcccaaagacttgtttcagcttgggctgcatctcaaagttctggaggcctccatgcacagatattaagagcttggggagttccagctgccaatctttcaccatgagatggagcagtgagtctggcttggtgtcataggatacacggatatacatggctttattggaatatccgccaccctggaattcaagaactccataggaatctgttgggtagctctgggtgtgcttggcaacagaccatttctcaggctgagtctccacctgtttgctttcctcttcatttttgctgggtgttgcacttggcagaggggggatatgctggttggtgaactggccacagcaacacctgttagagtctttcatgctaggaattacaaagatacattcccgtttgcaaaaggttttctctatccaagatttctgaccctgccacagcagtggaatggagagggcacagctcaggctctttcagcctcctccttggccagggcaggg

SEQ ID NO: 15650 - RNA, 5519 nt, Homo sapiens
  source 1..5519: mol_type = other RNA
gctgggattacaggcatgagccactgtgcccagctagttgcttacttcttaagtgacctaatggtgacttcagtgctcgagggcacttcctaggctatttggtggccctcagtaataaagagattgtataatcttgtatactgattagccaatttatcttcgttacagtatcatcactttcatttgatactactgcaactgaaaaaactaagcctactaacatatgctaacaaaatactacttttagtgcattaaattgtaaatcaagtctgaatttccaaaattttttaaggaaaatgtttttagaaattgatgatgtttagatggccaagatgacacccattagtggttctgactgttaaaaaaaaaaattaaagaaacaaaacagactagcattcagtttctgtggaagctttctctttcttaacctttttttcttctgctgtcattccagacacaattactaagctgcttacactactggcatgtccagatctgtctaactttccctgaatggatttcacattcctaggatgtccatgtaaactttttgacctgagagatgggaatcccaaagtttgatctggcttcacagacagtaagttttccatcccatttctgtcagtaatggttagggacaagcgagggattcgaggaattgcttcagcgacatggtgttcatcttgcatatctgcaaactgctctttatgctcagcttgcactgcagcttccgacacaatgtaaggaatatctgtgctatgagagcgcgtgatcttttgaacttggcattgccattccgtcgtcaattgctggtccgtgattgaactgtactctacatcctggttaaccccaccgaccagctttcttccccgggaatagacgaagcttctggacttcattgttttacaagcattgatcgtttcatcggggaaatagcgtgtaattttggtttcttccaggggataggaaatagtgccttctatatttgtcgtttccactgttagctgagtgttttgaacatctgatttgtcctgtccatgtatcacatctgttttatttaaacttggggaaatagtttcttcttttttagagtctgtctgtctttcatcatcttcctttgaaatcccaatatctggacctaattttgactcttcagcgttctttaagtcatctactgcaaggtgactgccatctggggttgctgatgtgcttgtgcccagtgaaaggtgaagactgttctgacattctgggactaggtgcgttttcacgtccttctcttcctttatacggaaggaacaggtttttttcctgactcctgtccctggtgacgtggagagagatgtatcctcaaataataactcttctccgttaaaatgatatcgatacaagctgtagccatcagcgctattgatgctgctttgccggagaagatacgttgcctcacattcagaagaagcccgggaccgtgcctggatcaggtcagacctgtcgattcccgcaagattttcaagagcattcaccattctgttagataattcttctagctgagcaagtcgaaggtcaacagtctgcagggaagttttcataaaagtttctctttcattgatttcttccaacctcattgacatattttcaactctttcagaagtgacccggatgcgctcgtcgctggacgactgctgctcatcctccttctcccggaagtgctcctgcacgcactgctcctcgaactcatgcagcctctttagctcctcgtcgctaaggaagagcttcaatccacgatcccgttcctcttggtccccttctctctttttcctgcagcggccgctgagacgcataatgatgatgtagatgtggcttaaaatgatcatcggtgggggcaggactggcctgtcatgaaatgtcataatcagctgatatcgctggaacttccacacctggttggatattgattttacttcaaagaaggtattgttgaacacagcaatcagcaggttcaccagcaggatgttggcgaccagtagatagcacgccatgagtgctggagtgagccaggcgccggggatacagggaggaagccgcttgccctcctcatcatataggttctcaccacaaggaggattaatttccatggcgtagaggtctatctggtctgcaaacacctctccatagatcatccagtagggcatgtagaagatgtttcgggccagtttccaagagggcttctcctctggatgcagaatggcttgacgggctactccgaaactcatgagcacgaccagcatgatgaccacaaagtacagcatgtcgatcatcatctttccaatcatcatcacgtatggccccagatacttgttgacaccaaagatgtccaggacacggatgtaccagaagatgatatccacacagtagatcacccggccatagcccatgtagggctggttctgtaggcgaagaattgctccaatcatgaatgtggaaatggccacgagatctgtgatgttccagtactcctgaagccaaactttgattttctggctgagtttgcctggttctgacatgaggatctctcgtatcttctctaacgccaggctcacgatgtaggagatgacgatccactcctggagggacggccagccatccatccgcaccaggatgacgtagttaaacagcagcaggtagcccaagtatgatattgtgtaaaaccagaacttgacaatgggcgcgttatagaattcacagatctttgttccgatgggaatacttctctgttttttgtgctcgttctcctcatccccctttcttgagccagcatctgcatttgcatccgtattttcctcttctttttctttgccatcctcattttccttggatgtttgatacgagaaatcatcatatgtgcgaaattccaaaaacaagatggtggggggtagaagaatccccatgataaccttcaggccggggttcttccgcatccgcagtcttcccatccacatatcggtcagcagcatctggctgcaggtgtgagcaatgaagtcccggtgtttggctgccacggccagtttgaggcaggtcgagttgctccagtttttcagctcgtaggtcaggagtttcatagcgatctgctcgtcatgcttataggactggtctaataactccaaagcaagctggccgaagtctttggaattgttatccaagtcctgggagatgtcatccaccagatcactctcggaggactcgtgggccatggccttgtagagcttgcaggccaccagggccttggccatgctctcttcccctcgctgccagaggaacactgccattttctggcgtttcatcagcactgcccacaccatcagctcgtggaagggatactggaaccgactcacggcagggtcgtccacatcaatgtcgatctcttcctcctttttcttctttttctttttcttccctttagctggaggctcatcatcttccattcccagaagtttaagagctttaggcctctttggtccaaacaagttgttgtaaagggtccgaaagtttttccgagtgtagttgcagcggtaggctcctcccatgaggtactccagcacgagcccgatgtctatgaggctgatgtggtaatcaggcggaaggttgctctttttcacatccctcaccagcagatgaagtgtgtttggtggacccagtcttgtgttataaagctcctccagcctcggaatggtcagaaagtgttgcatgttcactccgttttcaatcaggagcttcacaaagtcgacacgatctaagactaaagcatctagcatcgcttgctccaaagcattcacccagttcagcagctctatcttccgggggtcagtttcttcctccacttcctctttcactttccctttcttcttgcctttcccttttcctcttcctcccttggtggtggccatgggtggcttcttctccttctccgtggctttgctgtccgtcgggggtgccaggcttcccaggggcggccagtggggcccaaagacaaagatctggcttcgtgctatgtccacgcggttccaagccagtgccaagctcagctgatctggagcagatacgtttgttcctttcagcagggcagttaaaattgccatctcgatgtcctgctggccctcagaacccattctgaacacagtgacgagttctttcttcttcatgcactccattataattgcaaacagctgatgtgattgtgccttattataattaaatgttttctgaatggtaactagaagctgctccctgagggactcatttattattccgccttcttcacagtacttgtgcgcaaaggacaggatgtccgaggcacgtccgctgccatcacaaatcaccacagggatgggaggctcttcttgcaggtattccaagacgatggacaccacgttagggcccccctccaccacgagacccacgaggggcacgccctgccccagtcttgtgttgatcttctgcagggagatgtgcttttccagcagccttcgcagcttcacctcggcgccatacttgcccagggtgccattgtcagccaggatgaagtgggtgtgggagttgttgagcacagagagcttacttagagggttggacatggtctggtacactcttgttacatcctttccaaccaggtcttccttattctccacgatgccccatggagcaattcctatagcacaaacccggcctctggacttggaggagtggtctttcaaggcatcccctacgtggctgataacacctgtgctgacacccccggtgaagatccaggccccggtggtcatagcagccttgatcaggcctttcccaaagacttgtttcagcttgggctgcatctcaaagttctggaggcctccatgcacagatattaagagcttggggagttccagctgccaatctttcaccatgagatggagcagtgagtctggcttggtgtcataggatacacggatatacatggctttattggaatatccgccaccctggaattcaagaactccataggaatctgttgggtagctctgggtgtgcttggcaacagaccatttctcaggctgagtctccacctgtttgctttcctcttcatttttgctgggtgttgcacttggcagaggggggatatgctggttggtgaactggccacagcaacacctgttagagtctttcatgctaggaattacaaagatacattcccgtttgcaaaaggttttctctatccaagatttctgacccttctgcgaccctgatgtggagctcttgagcgagccccgcttgaaggagctcatctctctcagtgagcctgtgagccaccctgctgactccctcgggtggccaggccagtggcacaggggctgccctccctgggtgggcaggagcggagccacacactcggcggcagccccacactcggcggcagccccacgcactgggcgagggggccgagatcctggggcgaggccggccggaggctggttcagcctaggagg

SEQ ID NO: 15651 - RNA, 6896 nt, Homo sapiens
  source 1..6896: mol_type = other RNA
gctgggattacaggcatgagccactgtgcccagctgaagtgtgatccttaacttcaccccttctcatgccctccatttccaatccatctccagtccagttgactccagctactcaattatttccacttatctcattccactacctttgaagctaccaccatctctaactacagtcatctcccaactaactggtctcctggcatctctctggttctcctccactaatttcaaaaaaagaaatttactgtgacagtgctcacaacactcccccttgctcttactaaagatgcttaccatagcctccaggtattgtatggcctgaggtctatctacatttccaggtgcaggacacaccatgtctccccactcccaaatttagtctccagactccatcctttttacagttctttaaaagcatcacaattcctccaaccactaggcatttgtatgtgctattccctctttccagaatgcaataccctccctctgcctagctagctaacttctatgtatctatgactgcagctcaaactttcctcatggactccctccacaagtgccaagcctgggccagattcttttgttatgtgctcacagaacgatgttccctttagcattcattgagtttgctgtttaattattcttgtcttgtttttgtttaattagtcctatctctaatactagacaaatgttccttaagatcacaggaaatataggactgtctctacataaaaactgttttatatccataatgcctaggacagtacctggcacacagtatatgctcaataaatttttgttgaatgaatgcaattatcattatattcctgatattagcaggtataatccagtttaagtttgggaacagaaagacaaaacggaccacatctaataaatccggtctcctttcttttattatttatttatttgagacagttttgctcttgttgcccaggctgcagtgcaatggcatgatcttggctcactgaaacctccgcctcccaagttcaagggattctccagcctcagcctcccaagtagctgggattacaggcatccaccaccacgcccagctaatttttttgtatttttagtagagatggggtttcaccatgttggccaggctggtctcgaactcctgacctcaggtgatccacccacctcagcctcccaaagtgttgggattacaggcgtgagccaccgtgcccggccaaggtctcctttcttttaatcaaactctcacctttggccattctgcagtcattcacccgacagtatttactgacggagtgaatacagagtgcttgattaatgttgctgctttgttattattattattattattgagatggagtcttgctctgttgcccaggctggagtgcagtggcgtgatctcggctcactgcaacctccgcctcccgggttcaagccattctcctgcctcagcctcccaagtagctgggactacaggcatgcaacaccacacctggctaatttttgtatttttagtagagacaaggtttcaccatattggccaggctggtcttgaactcctgacctcaggtgatctgcccacctcagcttcccaaagtgctgggattacaggcgtgagccaccatacccaacctaatgtttctgctttgaaatacaatttcaaaaagtcattaataggttgaaaacagcaagattttaaaagtattttaaaaagtgaaacagaagaatgcttacttcatttcacagagatagatttctcctttatgttatttctaaaaggagatggaattttgtttcattcatttctgcttatttggacaggccaaatatgaacagctgaacacgtcagcgttaccatgcatatgttacacagatgccatccttcttccatcagctctcatatgcaatacagaagtaaaaagaggttctctttatttttaaaaggtaaaaattgaaattcagtcacttaacacagaataaacaataattacaattacactggtaacaaaggacagcaagcatgttttctttgaaagcactgtatctggtttgtctccgtgcttggtcctagtatctggcatattttccccagagttttcttttcagtgggatgattatcttcggggcaaaaaagtttatcagactcaagttttagcagtacttattttattcatttatatacatgtaaccccatcctgtcttactccaatcttcttactgccttcctactgacacatatattatataacaccctccccaagttctatttacggttaaaaatttctttttttttttctttttttgagacagagtttcactctcgtcacccaggctggtgtgcaatggcgcagtctcggctcactgcaacctccgactccctggttcaagtgattctcctgtctcagcctcccgagtagctggaattacaggcgcccgccaccatgcccagctaatttttgtatttttagtagagacagtgtttcgccatgttggccaggctggtctcaaactcctgacctcaggtgatccacccgccttggcctctcaaagtgctgggattataggcgtaagccactgcgcccagcctacagttacgaatttctaaatggcacaaataaactcagctgttctcagtgcagacgtcaaatcctcactgtgctgaaacattttcctcagcttttgggaaataattacaatttaaacatacacagagaatgtttcttagacaaacataatacccgaggcttatctggtaaaaactaattgctctgtccttagcacaaaaaatatatatctttgtaaaatgagaagaaccaaagaatatttaaaacaaagaaggaagccacacgtactaattacacaagagactgactgacaaactggaattctccaaaacagattttcagcgaggcttctcatttcagagtccaggaaaaaaaaatcctaaaaaccccaaaggtatattatatgtgtgtatatatatttttattgtgttaaaaaacacaaaacataaaatttactgtcttatcaaaaggtatattttgtcgctcttccctttttttttttttttttttcccgagacagagtccagtctgtcgcccaggctgaagtgcagtggcatgatctcggctcactgcaacctgcatcttctgggctcaagcaatcctcccacctcagcctcctgagtagatggagctacaggcacgtgccactaggcccggctaatttttgtattttttgcagacagggttttgccatgttgcccgggctggtctttgttctcctaagagttgttttctccatgaaagttgataaataacatttagaaaatgaattattacaagagtaatgatatgtctcaatttattatatgaaattatcaacaactgcttttaatattcagatgtcaagaagatgaaaagcagaaatacattttgcaaacatgtagcactccataaatggaaatcatgtatttcctctaatatcccaatttttctatattgggatcttatatggctgtttctatatggctattttgtcccaacttgctgtacaagaattttccccagccaccttagaaaggttggatgtagttcactccaagtttgcagttcactccaagtgtttcagtaccacagaaagctccatggaagcctcaaatgtacgggctaggcaatagaagcagggaggtaggattaagaaattactggccaggtgtggtggctcaggcctgtaatcccagcacttcgagaggctgaggcagacagatggcttgagctcaagagtttgagatcagcctgagcaacatggcaaaactctgtctctacaaaaaatataaaaatcagccaggtatgttggtgtgcacctgtagtcccagctactggggaggttgaggcaggaggattgcttgagcccaggaggctgaggctgcagtgagccatgattgtgccactgcattccagcctggtcgactgtaagacaaaaaataagaaaataaaaaatttaccaatataaaatgctcaaacagctaacaaacatgttcaattccatttatagtcttttctttgagccatttaaacatagggctattttttttttttttttttgagatggagtttcactcttgttgcccaggctggagagcaatggcatgatctcggctcaccacaacctctgcctcctgggttcaagcgattctcctgcctcagcctcccgagcagctgggattacaggcatgtgccaccatgcctggctaattttgtatttttagtagagacgggattcctccatgttggtcagactggtcttgaactcccaacctcaggtgatctgcctgcctcaaccttccaaagtgctgggattacaggtgtgagccactgagattggctgccgttttgttttttaactccatatagtttctatagttcactgaaaactcaaagagatgacctataaatgtatgaataatgtatgatttcttacatcaattttctactagaaaaaaatcatacttttagaattggattttgtcttacagtcatctttattatactttataaatgagatttcatttatataaatcaggaagctaaactaaaatagaaacactagatttaaattctgatttgaatactctgatcaaaataacaaatctcacactgggaaaccatctatcagcaagcagagagctactgtgtgtccttccttagaagagtttgaacaccgagaacccacagcatatttgcagtacagtaacagcaattcctttgtcattatcacagaactttaattttcatatactttgctgggaccaaccaaaccatcccatatatataaccatatccatatatatatatatatatatcccacatatatatgggatggtatatatatacacatgtatatgtatgtgtgtgtgtatatatgtgtatatatgtatacacacacacacacacacatatatatatatatacacacacacacatatatatatggagagagagagagagacagtgtcttgctctgtcgcccaggctggagtgcagtggtacgatcttggctcattgcaacctccgcctcccaggctcaagcgattctcatgtctcagtctcccaagtagctgggattacaggtgtgcaccaccacaccaggctaaccattccatacattttatacaatcatttttaaaaagaagcatgaaccatttcggttttagagaattaagtttttttaaaaaagagactcttaaaaaaaagtcattatatgaataaaatctgctttgtgttaattccgacaaatcattccatcattgagtctgtcaccaattttttttttttgaaatggagtttcgctcttgttgcccaggctggagtgcaatggtacgatctcggctcactgcaaccgccgcctcccgggttcaagtgattctcctgcctcagcctcccgagtagctgggattacaggcatgcgccaccacgcctggctaattttgtattattagttgagacagggtttctccatgttggtcaggctggtctcgaactcctgacctcaagtgatccgctggccttggcctcccaaagtgctgggattacaggcgtgagccaccgtgcctggcccaattttttttttttaataacttgcacacttaacaatattttttatcttcttgggacaacattcttttctccacaaaaacccaattaaggacgttgtgccagtttactcctacttccttcctgttcactgagcttaaagtgggtataggcgagaatgccaaataatgtacataaaatgccaagggcctgattaatggacagtggatccttaaataaaacatatcctccgaataaagtaatgcagaacttgaagtgtccgaacatgttataggtgacaggtgaagtgttcccaatgatccaataaattgataagttcaccatgaaagctattactccagatagcagcaccataagcaaagcagaaactgaccagggaccaaatattcctccttctccaaacactggctcaaagaagggcacagcaaccagcaacatggcagatgacatcggagcctggtagtacagcagctgcattgagttcacttgtaattcatgctgtttggctcctacccaaaacaggtaggtatttggtgagcatcacacacccaagtttctctgtctcctttcttctcttcaccttgagtcagacaacttatgcaattatgctttcttcccaacagtctattgtctctatactgtattttctaaaccttggaatacagcttcaaaatttatgaaatcagcgtgagctggattctggtggagaaggttttctggtagcagaaggtctggatggctatgatcaccggcgtggtcatggccttggccagctgataggtgcctatggtgttgttctgcagagaaaggttagtgaagaccacaaagccacagaagctgagggccaggaggaggagcctggagggcggcagacttttgggggcaaagatgtccagcttctggcagatatacaagcccagccaggtgaccacgaagtgcaccagggtcaggctcatgttggggaagccgtggtacacataaatccatttgttgaggaacacaatgcagatggacaccagcaggttgaacaggagcccggcggcgattcgccagtggccccgcactcggtccaccagcaatgccatgatccccgcgaagctggggccgtctagcctcggaaggggcgccgggcctgtctccggctgcccttctactccaccgccgcgtcctcgcagacgccgacctcaccgtctgacccaggagtggcatgcacagatcaaccccgggcgagtagcactcttaacagaggacacacaccccgccgccgccctgtaagccagctaggac

SEQ ID NO: 15652 - RNA, 6899 nt, Homo sapiens
  source 1..6899: mol_type = other RNA
gctgggattacaggcatgagccactgtgcccagctgaagtgtgatccttaacttcaccccttctcatgccctccatttccaatccatctccagtccagttgactccagctactcaattatttccacttatctcattccactacctttgaagctaccaccatctctaactacagtcatctcccaactaactggtctcctggcatctctctggttctcctccactaatttcaaaaaaagaaatttactgtgacagtgctcacaacactcccccttgctcttactaaagatgcttaccatagcctccaggtattgtatggcctgaggtctatctacatttccaggtgcaggacacaccatgtctccccactcccaaatttagtctccagactccatcctttttacagttctttaaaagcatcacaattcctccaaccactaggcatttgtatgtgctattccctctttccagaatgcaataccctccctctgcctagctagctaacttctatgtatctatgactgcagctcaaactttcctcatggactccctccacaagtgccaagcctgggccagattcttttgttatgtgctcacagaacgatgttccctttagcattcattgagtttgctgtttaattattcttgtcttgtttttgtttaattagtcctatctctaatactagacaaatgttccttaagatcacaggaaatataggactgtctctacataaaaactgttttatatccataatgcctaggacagtacctggcacacagtatatgctcaataaatttttgttgaatgaatgcaattatcattatattcctgatattagcaggtataatccagtttaagtttgggaacagaaagacaaaacggaccacatctaataaatccggtctcctttcttttattatttatttatttgagacagttttgctcttgttgcccaggctgcagtgcaatggcatgatcttggctcactgaaacctccgcctcccaagttcaagggattctccagcctcagcctcccaagtagctgggattacaggcatccaccaccacgcccagctaatttttttgtatttttagtagagatggggtttcaccatgttggccaggctggtctcgaactcctgacctcaggtgatccacccacctcagcctcccaaagtgttgggattacaggcgtgagccaccgtgcccggccaaggtctcctttcttttaatcaaactctcacctttggccattctgcagtcattcacccgacagtatttactgacggagtgaatacagagtgcttgattaatgttgctgctttgttattattattattattattgagatggagtcttgctctgttgcccaggctggagtgcagtggcgtgatctcggctcactgcaacctccgcctcccgggttcaagccattctcctgcctcagcctcccaagtagctgggactacaggcatgcaacaccacacctggctaatttttgtatttttagtagagacaaggtttcaccatattggccaggctggtcttgaactcctgacctcaggtgatctgcccacctcagcttcccaaagtgctgggattacaggcgtgagccaccatacccaacctaatgtttctgctttgaaatacaatttcaaaaagtcattaataggttgaaaacagcaagattttaaaagtattttaaaaagtgaaacagaagaatgcttacttcatttcacagagatagatttctcctttatgttatttctaaaaggagatggaattttgtttcattcatttctgcttatttggacaggccaaatatgaacagctgaacacgtcagcgttaccatgcatatgttacacagatgccatccttcttccatcagctctcatatgcaatacagaagtaaaaagaggttctctttatttttaaaaggtaaaaattgaaattcagtcacttaacacagaataaacaataattacaattacactggtaacaaaggacagcaagcatgttttctttgaaagcactgtatctggtttgtctccgtgcttggtcctagtatctggcatattttccccagagttttcttttcagtgggatgattatcttcggggcaaaaaagtttatcagactcaagttttagcagtacttattttattcatttatatacatgtaaccccatcctgtcttactccaatcttcttactgccttcctactgacacatatattatataacaccctccccaagttctatttacggttaaaaatttctttttttttttctttttttgagacagagtttcactctcgtcacccaggctggtgtgcaatggcgcagtctcggctcactgcaacctccgactccctggttcaagtgattctcctgtctcagcctcccgagtagctggaattacaggcgcccgccaccatgcccagctaatttttgtatttttagtagagacagtgtttcgccatgttggccaggctggtctcaaactcctgacctcaggtgatccacccgccttggcctctcaaagtgctgggattataggcgtaagccactgcgcccagcctacagttacgaatttctaaatggcacaaataaactcagctgttctcagtgcagacgtcaaatcctcactgtgctgaaacattttcctcagcttttgggaaataattacaatttaaacatacacagagaatgtttcttagacaaacataatacccgaggcttatctggtaaaaactaattgctctgtccttagcacaaaaaatatatatctttgtaaaatgagaagaaccaaagaatatttaaaacaaagaaggaagccacacgtactaattacacaagagactgactgacaaactggaattctccaaaacagattttcagcgaggcttctcatttcagagtccaggaaaaaaaaatcctaaaaaccccaaaggtatattatatgtgtgtatatatatttttattgtgttaaaaaacacaaaacataaaatttactgtcttatcaaaaggtatattttgtcgctcttccctttttttttttttttttttcccgagacagagtccagtctgtcgcccaggctgaagtgcagtggcatgatctcggctcactgcaacctgcatcttctgggctcaagcaatcctcccacctcagcctcctgagtagatggagctacaggcacgtgccactaggcccggctaatttttgtattttttgcagacagggttttgccatgttgcccgggctggtctttgttctcctaagagttgttttctccatgaaagttgataaataacatttagaaaatgaattattacaagagtaatgatatgtctcaatttattatatgaaattatcaacaactgcttttaatattcagatgtcaagaagatgaaaagcagaaatacattttgcaaacatgtagcactccataaatggaaatcatgtatttcctctaatatcccaatttttctatattgggatcttatatggctgtttctatatggctattttgtcccaacttgctgtacaagaattttccccagccaccttagaaaggttggatgtagttcactccaagtttgcagttcactccaagtgtttcagtaccacagaaagctccatggaagcctcaaatgtacgggctaggcaatagaagcagggaggtaggattaagaaattactggccaggtgtggtggctcaggcctgtaatcccagcacttcgagaggctgaggcagacagatggcttgagctcaagagtttgagatcagcctgagcaacatggcaaaactctgtctctacaaaaaatataaaaatcagccaggtatgttggtgtgcacctgtagtcccagctactggggaggttgaggcaggaggattgcttgagcccaggaggctgaggctgcagtgagccatgattgtgccactgcattccagcctggtcgactgtaagacaaaaaataagaaaataaaaaatttaccaatataaaatgctcaaacagctaacaaacatgttcaattccatttatagtcttttctttgagccatttaaacatagggctattttttttttttttttttgagatggagtttcactcttgttgcccaggctggagagcaatggcatgatctcggctcaccacaacctctgcctcctgggttcaagcgattctcctgcctcagcctcccgagcagctgggattacaggcatgtgccaccatgcctggctaattttgtatttttagtagagacgggattcctccatgttggtcagactggtcttgaactcccaacctcaggtgatctgcctgcctcaaccttccaaagtgctgggattacaggtgtgagccactgagattggctgccgttttgttttttaactccatatagtttctatagttcactgaaaactcaaagagatgacctataaatgtatgaataatgtatgatttcttacatcaattttctactagaaaaaaatcatacttttagaattggattttgtcttacagtcatctttattatactttataaatgagatttcatttatataaatcaggaagctaaactaaaatagaaacactagatttaaattctgatttgaatactctgatcaaaataacaaatctcacactgggaaaccatctatcagcaagcagagagctactgtgtgtccttccttagaagagtttgaacaccgagaacccacagcatatttgcagtacagtaacagcaattcctttgtcattatcacagaactttaattttcatatactttgctgggaccaaccaaaccatcccatatatataaccatatccatatatatatatatatatatcccacatatatatgggatggtatatatatacacatgtatatgtatgtgtgtgtgtatatatgtgtatatatgtatacacacacacacacacacatatatatatatatacacacacacacatatatatatggagagagagagagagacagtgtcttgctctgtcgcccaggctggagtgcagtggtacgatcttggctcattgcaacctccgcctcccaggctcaagcgattctcatgtctcagtctcccaagtagctgggattacaggtgtgcaccaccacaccaggctaaccattccatacattttatacaatcatttttaaaaagaagcatgaaccatttcggttttagagaattaagtttttttaaaaaagagactcttaaaaaaaagtcattatatgaataaaatctgctttgtgttaattccgacaaatcattccatcattgagtctgtcaccaattttttttttttgaaatggagtttcgctcttgttgcccaggctggagtgcaatggtacgatctcggctcactgcaaccgccgcctcccgggttcaagtgattctcctgcctcagcctcccgagtagctgggattacaggcatgcgccaccacgcctggctaattttgtattattagttgagacagggtttctccatgttggtcaggctggtctcgaactcctgacctcaagtgatccgctggccttggcctcccaaagtgctgggattacaggcgtgagccaccgtgcctggcccaattttttttttttaataacttgcacacttaacaatattttttatcttcttgggacaacattcttttctccacaaaaacccaattaaggacgttgtgccagtttactcctacttccttcctgttcactgagcttaaagtgggtataggcgagaatgccaaataatgtacataaaatgccaagggcctgattaatggacagtggatccttaaataaaacatatcctccgaataaagtaatgcagaacttgaagtgtccgaacatgttataggtgacaggtgaagtgttcccaatgatccaataaattgataagttcaccatgaaagctattactccagatagcagcaccataagcaaagcagaaactgaccagggaccaaatattcctccttctccaaacactggctcaaagaagggcacagcaaccagcaacatggcagatgacatcggagcctggtagtacagcagctgcattgagttcacttgtaattcatgctgtttggctcctacccaaaacaggtaggtatttggtgagcatcacacacccaagtttctctgtctcctttcttctcttcaccttgagtcagacaacttatgcaattatgctttcttcccaacagtctattgtctctatactgtattttctaaaccttggaatacagcttcaaaatttatgaaatctgcagcgtgagctggattctggtggagaaggttttctggtagcagaaggtctggatggctatgatcaccggcgtggtcatggccttggccagctgataggtgcctatggtgttgttctgcagagaaaggttagtgaagaccacaaagccacagaagctgagggccaggaggaggagcctggagggcggcagacttttgggggcaaagatgtccagcttctggcagatatacaagcccagccaggtgaccacgaagtgcaccagggtcaggctcatgttggggaagccgtggtacacataaatccatttgttgaggaacacaatgcagatggacaccagcaggttgaacaggagcccggcggcgattcgccagtggccccgcactcggtccaccagcaatgccatgatccccgcgaagctggggccgtctagcctcggaaggggcgccgggcctgtctccggctgcccttctactccaccgccgcgtcctcgcagacgccgacctcaccgtctgacccaggagtggcatgcacagatcaaccccgggcgagtagcactcttaacagaggacacacaccccgccgccgccctgtaagccagctaggac

SEQ ID NO: 15653 - RNA, 6840 nt, Homo sapiens
  source 1..6840: mol_type = other RNA
gctgggattacaggcatgagccactgtgcccagctgaagtgtgatccttaacttcaccccttctcatgccctccatttccaatccatctccagtccagttgactccagctactcaattatttccacttatctcattccactacctttgaagctaccaccatctctaactacagtcatctcccaactaactggtctcctggcatctctctggttctcctccactaatttcaaaaaaagaaatttactgtgacagtgctcacaacactcccccttgctcttactaaagatgcttaccatagcctccaggtattgtatggcctgaggtctatctacatttccaggtgcaggacacaccatgtctccccactcccaaatttagtctccagactccatcctttttacagttctttaaaagcatcacaattcctccaaccactaggcatttgtatgtgctattccctctttccagaatgcaataccctccctctgcctagctagctaacttctatgtatctatgactgcagctcaaactttcctcatggactccctccacaagtgccaagcctgggccagattcttttgttatgtgctcacagaacgatgttccctttagcattcattgagtttgctgtttaattattcttgtcttgtttttgtttaattagtcctatctctaatactagacaaatgttccttaagatcacaggaaatataggactgtctctacataaaaactgttttatatccataatgcctaggacagtacctggcacacagtatatgctcaataaatttttgttgaatgaatgcaattatcattatattcctgatattagcaggtataatccagtttaagtttgggaacagaaagacaaaacggaccacatctaataaatccggtctcctttcttttattatttatttatttgagacagttttgctcttgttgcccaggctgcagtgcaatggcatgatcttggctcactgaaacctccgcctcccaagttcaagggattctccagcctcagcctcccaagtagctgggattacaggcatccaccaccacgcccagctaatttttttgtatttttagtagagatggggtttcaccatgttggccaggctggtctcgaactcctgacctcaggtgatccacccacctcagcctcccaaagtgttgggattacaggcgtgagccaccgtgcccggccaaggtctcctttcttttaatcaaactctcacctttggccattctgcagtcattcacccgacagtatttactgacggagtgaatacagagtgcttgattaatgttgctgctttgttattattattattattattgagatggagtcttgctctgttgcccaggctggagtgcagtggcgtgatctcggctcactgcaacctccgcctcccgggttcaagccattctcctgcctcagcctcccaagtagctgggactacaggcatgcaacaccacacctggctaatttttgtatttttagtagagacaaggtttcaccatattggccaggctggtcttgaactcctgacctcaggtgatctgcccacctcagcttcccaaagtgctgggattacaggcgtgagccaccatacccaacctaatgtttctgctttgaaatacaatttcaaaaagtcattaataggttgaaaacagcaagattttaaaagtattttaaaaagtgaaacagaagaatgcttacttcatttcacagagatagatttctcctttatgttatttctaaaaggagatggaattttgtttcattcatttctgcttatttggacaggccaaatatgaacagctgaacacgtcagcgttaccatgcatatgttacacagatgccatccttcttccatcagctctcatatgcaatacagaagtaaaaagaggttctctttatttttaaaaggtaaaaattgaaattcagtcacttaacacagaataaacaataattacaattacactggtaacaaaggacagcaagcatgttttctttgaaagcactgtatctggtttgtctccgtgcttggtcctagtatctggcatattttccccagagttttcttttcagtgggatgattatcttcggggcaaaaaagtttatcagactcaagttttagcagtacttattttattcatttatatacatgtaaccccatcctgtcttactccaatcttcttactgccttcctactgacacatatattatataacaccctccccaagttctatttacggttaaaaatttctttttttttttctttttttgagacagagtttcactctcgtcacccaggctggtgtgcaatggcgcagtctcggctcactgcaacctccgactccctggttcaagtgattctcctgtctcagcctcccgagtagctggaattacaggcgcccgccaccatgcccagctaatttttgtatttttagtagagacagtgtttcgccatgttggccaggctggtctcaaactcctgacctcaggtgatccacccgccttggcctctcaaagtgctgggattataggcgtaagccactgcgcccagcctacagttacgaatttctaaatggcacaaataaactcagctgttctcagtgcagacgtcaaatcctcactgtgctgaaacattttcctcagcttttgggaaataattacaatttaaacatacacagagaatgtttcttagacaaacataatacccgaggcttatctggtaaaaactaattgctctgtccttagcacaaaaaatatatatctttgtaaaatgagaagaaccaaagaatatttaaaacaaagaaggaagccacacgtactaattacacaagagactgactgacaaactggaattctccaaaacagattttcagcgaggcttctcatttcagagtccaggaaaaaaaaatcctaaaaaccccaaaggtatattatatgtgtgtatatatatttttattgtgttaaaaaacacaaaacataaaatttactgtcttatcaaaaggtatattttgtcgctcttccctttttttttttttttttttcccgagacagagtccagtctgtcgcccaggctgaagtgcagtggcatgatctcggctcactgcaacctgcatcttctgggctcaagcaatcctcccacctcagcctcctgagtagatggagctacaggcacgtgccactaggcccggctaatttttgtattttttgcagacagggttttgccatgttgcccgggctggtctttgttctcctaagagttgttttctccatgaaagttgataaataacatttagaaaatgaattattacaagagtaatgatatgtctcaatttattatatgaaattatcaacaactgcttttaatattcagatgtcaagaagatgaaaagcagaaatacattttgcaaacatgtagcactccataaatggaaatcatgtatttcctctaatatcccaatttttctatattgggatcttatatggctgtttctatatggctattttgtcccaacttgctgtacaagaattttccccagccaccttagaaaggttggatgtagttcactccaagtttgcagttcactccaagtgtttcagtaccacagaaagctccatggaagcctcaaatgtacgggctaggcaatagaagcagggaggtaggattaagaaattactggccaggtgtggtggctcaggcctgtaatcccagcacttcgagaggctgaggcagacagatggcttgagctcaagagtttgagatcagcctgagcaacatggcaaaactctgtctctacaaaaaatataaaaatcagccaggtatgttggtgtgcacctgtagtcccagctactggggaggttgaggcaggaggattgcttgagcccaggaggctgaggctgcagtgagccatgattgtgccactgcattccagcctggtcgactgtaagacaaaaaataagaaaataaaaaatttaccaatataaaatgctcaaacagctaacaaacatgttcaattccatttatagtcttttctttgagccatttaaacatagggctattttttttttttttttttgagatggagtttcactcttgttgcccaggctggagagcaatggcatgatctcggctcaccacaacctctgcctcctgggttcaagcgattctcctgcctcagcctcccgagcagctgggattacaggcatgtgccaccatgcctggctaattttgtatttttagtagagacgggattcctccatgttggtcagactggtcttgaactcccaacctcaggtgatctgcctgcctcaaccttccaaagtgctgggattacaggtgtgagccactgagattggctgccgttttgttttttaactccatatagtttctatagttcactgaaaactcaaagagatgacctataaatgtatgaataatgtatgatttcttacatcaattttctactagaaaaaaatcatacttttagaattggattttgtcttacagtcatctttattatactttataaatgagatttcatttatataaatcaggaagctaaactaaaatagaaacactagatttaaattctgatttgaatactctgatcaaaataacaaatctcacactgggaaaccatctatcagcaagcagagagctactgtgtgtccttccttagaagagtttgaacaccgagaacccacagcatatttgcagtacagtaacagcaattcctttgtcattatcacagaactttaattttcatatactttgctgggaccaaccaaaccatcccatatatataaccatatccatatatatatatatatatatcccacatatatatgggatggtatatatatacacatgtatatgtatgtgtgtgtgtatatatgtgtatatatgtatacacacacacacacacacatatatatatatatacacacacacacatatatatatggagagagagagagagacagtgtcttgctctgtcgcccaggctggagtgcagtggtacgatcttggctcattgcaacctccgcctcccaggctcaagcgattctcatgtctcagtctcccaagtagctgggattacaggtgtgcaccaccacaccaggctaaccattccatacattttatacaatcatttttaaaaagaagcatgaaccatttcggttttagagaattaagtttttttaaaaaagagactcttaaaaaaaagtcattatatgaataaaatctgctttgtgttaattccgacaaatcattccatcattgagtctgtcaccaattttttttttttgaaatggagtttcgctcttgttgcccaggctggagtgcaatggtacgatctcggctcactgcaaccgccgcctcccgggttcaagtgattctcctgcctcagcctcccgagtagctgggattacaggcatgcgccaccacgcctggctaattttgtattattagttgagacagggtttctccatgttggtcaggctggtctcgaactcctgacctcaagtgatccgctggccttggcctcccaaagtgctgggattacaggcgtgagccaccgtgcctggcccaattttttttttttaataacttgcacacttaacaatattttttatcttcttgggacaacattcttttctccacaaaaacccaattaaggacgttgtgccagtttactcctacttccttcctgttcactgagcttaaagtgggtataggcgagaatgccaaataatgtacataaaatgccaagggcctgattaatggacagtggatccttaaataaaacatatcctccgaataaagtaatgcagaacttgaagtgtccgaacatgttataggtgacaggtgaagtgttcccaatgatccaataaattgataagttcaccatgaaagctattactccagatagcagcaccataagcaaagcagaaactgaccagggaccaaatattcctccttctccaaacactggctcaaagaagggcacagcaaccagcaacatggcagatgacatcggagcctggtagtacagcagctgcattgagttcacttgtaattcatgctgtttggctcctacccacacttgataaagggatgtaactaaaacaccaagagcagcaaacaccattccaaggaaattaaacttcacatcgtaataagaatttaggattacacctaaagttataggaatcagcgtgagctggattctggtggagaaggttttctggtagcagaaggtctggatggctatgatcaccggcgtggtcatggccttggccagctgataggtgcctatggtgttgttctgcagagaaaggttagtgaagaccacaaagccacagaagctgagggccaggaggaggagcctggagggcggcagacttttgggggcaaagatgtccagcttctggcagatatacaagcccagccaggtgaccacgaagtgcaccagggtcaggctcatgttggggaagccgtggtacacataaatccatttgttgaggaacacaatgcagatggacaccagcaggttgaacaggagcccggcggcgattcgccagtggccccgcactcggtccaccagcaatgccatgatccccgcgaagctggggccgtctagcctcggaaggggcgccgggcctgtctccggctgcccttctactccaccgccgcgtcctcgcagacgccgacctcaccgtctgacccaggagtggcatgcacagatcaaccccgggcgagtagcactcttaacagaggacacacaccccgccgccgccctgtaagccagctaggac

SEQ ID NO: 15654 - RNA, 6729 nt, Homo sapiens
  source 1..6729: mol_type = other RNA
gctgggattacaggcatgagccactgtgcccagctgaagtgtgatccttaacttcaccccttctcatgccctccatttccaatccatctccagtccagttgactccagctactcaattatttccacttatctcattccactacctttgaagctaccaccatctctaactacagtcatctcccaactaactggtctcctggcatctctctggttctcctccactaatttcaaaaaaagaaatttactgtgacagtgctcacaacactcccccttgctcttactaaagatgcttaccatagcctccaggtattgtatggcctgaggtctatctacatttccaggtgcaggacacaccatgtctccccactcccaaatttagtctccagactccatcctttttacagttctttaaaagcatcacaattcctccaaccactaggcatttgtatgtgctattccctctttccagaatgcaataccctccctctgcctagctagctaacttctatgtatctatgactgcagctcaaactttcctcatggactccctccacaagtgccaagcctgggccagattcttttgttatgtgctcacagaacgatgttccctttagcattcattgagtttgctgtttaattattcttgtcttgtttttgtttaattagtcctatctctaatactagacaaatgttccttaagatcacaggaaatataggactgtctctacataaaaactgttttatatccataatgcctaggacagtacctggcacacagtatatgctcaataaatttttgttgaatgaatgcaattatcattatattcctgatattagcaggtataatccagtttaagtttgggaacagaaagacaaaacggaccacatctaataaatccggtctcctttcttttattatttatttatttgagacagttttgctcttgttgcccaggctgcagtgcaatggcatgatcttggctcactgaaacctccgcctcccaagttcaagggattctccagcctcagcctcccaagtagctgggattacaggcatccaccaccacgcccagctaatttttttgtatttttagtagagatggggtttcaccatgttggccaggctggtctcgaactcctgacctcaggtgatccacccacctcagcctcccaaagtgttgggattacaggcgtgagccaccgtgcccggccaaggtctcctttcttttaatcaaactctcacctttggccattctgcagtcattcacccgacagtatttactgacggagtgaatacagagtgcttgattaatgttgctgctttgttattattattattattattgagatggagtcttgctctgttgcccaggctggagtgcagtggcgtgatctcggctcactgcaacctccgcctcccgggttcaagccattctcctgcctcagcctcccaagtagctgggactacaggcatgcaacaccacacctggctaatttttgtatttttagtagagacaaggtttcaccatattggccaggctggtcttgaactcctgacctcaggtgatctgcccacctcagcttcccaaagtgctgggattacaggcgtgagccaccatacccaacctaatgtttctgctttgaaatacaatttcaaaaagtcattaataggttgaaaacagcaagattttaaaagtattttaaaaagtgaaacagaagaatgcttacttcatttcacagagatagatttctcctttatgttatttctaaaaggagatggaattttgtttcattcatttctgcttatttggacaggccaaatatgaacagctgaacacgtcagcgttaccatgcatatgttacacagatgccatccttcttccatcagctctcatatgcaatacagaagtaaaaagaggttctctttatttttaaaaggtaaaaattgaaattcagtcacttaacacagaataaacaataattacaattacactggtaacaaaggacagcaagcatgttttctttgaaagcactgtatctggtttgtctccgtgcttggtcctagtatctggcatattttccccagagttttcttttcagtgggatgattatcttcggggcaaaaaagtttatcagactcaagttttagcagtacttattttattcatttatatacatgtaaccccatcctgtcttactccaatcttcttactgccttcctactgacacatatattatataacaccctccccaagttctatttacggttaaaaatttctttttttttttctttttttgagacagagtttcactctcgtcacccaggctggtgtgcaatggcgcagtctcggctcactgcaacctccgactccctggttcaagtgattctcctgtctcagcctcccgagtagctggaattacaggcgcccgccaccatgcccagctaatttttgtatttttagtagagacagtgtttcgccatgttggccaggctggtctcaaactcctgacctcaggtgatccacccgccttggcctctcaaagtgctgggattataggcgtaagccactgcgcccagcctacagttacgaatttctaaatggcacaaataaactcagctgttctcagtgcagacgtcaaatcctcactgtgctgaaacattttcctcagcttttgggaaataattacaatttaaacatacacagagaatgtttcttagacaaacataatacccgaggcttatctggtaaaaactaattgctctgtccttagcacaaaaaatatatatctttgtaaaatgagaagaaccaaagaatatttaaaacaaagaaggaagccacacgtactaattacacaagagactgactgacaaactggaattctccaaaacagattttcagcgaggcttctcatttcagagtccaggaaaaaaaaatcctaaaaaccccaaaggtatattatatgtgtgtatatatatttttattgtgttaaaaaacacaaaacataaaatttactgtcttatcaaaaggtatattttgtcgctcttccctttttttttttttttttttcccgagacagagtccagtctgtcgcccaggctgaagtgcagtggcatgatctcggctcactgcaacctgcatcttctgggctcaagcaatcctcccacctcagcctcctgagtagatggagctacaggcacgtgccactaggcccggctaatttttgtattttttgcagacagggttttgccatgttgcccgggctggtctttgttctcctaagagttgttttctccatgaaagttgataaataacatttagaaaatgaattattacaagagtaatgatatgtctcaatttattatatgaaattatcaacaactgcttttaatattcagatgtcaagaagatgaaaagcagaaatacattttgcaaacatgtagcactccataaatggaaatcatgtatttcctctaatatcccaatttttctatattgggatcttatatggctgtttctatatggctattttgtcccaacttgctgtacaagaattttccccagccaccttagaaaggttggatgtagttcactccaagtttgcagttcactccaagtgtttcagtaccacagaaagctccatggaagcctcaaatgtacgggctaggcaatagaagcagggaggtaggattaagaaattactggccaggtgtggtggctcaggcctgtaatcccagcacttcgagaggctgaggcagacagatggcttgagctcaagagtttgagatcagcctgagcaacatggcaaaactctgtctctacaaaaaatataaaaatcagccaggtatgttggtgtgcacctgtagtcccagctactggggaggttgaggcaggaggattgcttgagcccaggaggctgaggctgcagtgagccatgattgtgccactgcattccagcctggtcgactgtaagacaaaaaataagaaaataaaaaatttaccaatataaaatgctcaaacagctaacaaacatgttcaattccatttatagtcttttctttgagccatttaaacatagggctattttttttttttttttttgagatggagtttcactcttgttgcccaggctggagagcaatggcatgatctcggctcaccacaacctctgcctcctgggttcaagcgattctcctgcctcagcctcccgagcagctgggattacaggcatgtgccaccatgcctggctaattttgtatttttagtagagacgggattcctccatgttggtcagactggtcttgaactcccaacctcaggtgatctgcctgcctcaaccttccaaagtgctgggattacaggtgtgagccactgagattggctgccgttttgttttttaactccatatagtttctatagttcactgaaaactcaaagagatgacctataaatgtatgaataatgtatgatttcttacatcaattttctactagaaaaaaatcatacttttagaattggattttgtcttacagtcatctttattatactttataaatgagatttcatttatataaatcaggaagctaaactaaaatagaaacactagatttaaattctgatttgaatactctgatcaaaataacaaatctcacactgggaaaccatctatcagcaagcagagagctactgtgtgtccttccttagaagagtttgaacaccgagaacccacagcatatttgcagtacagtaacagcaattcctttgtcattatcacagaactttaattttcatatactttgctgggaccaaccaaaccatcccatatatataaccatatccatatatatatatatatatatcccacatatatatgggatggtatatatatacacatgtatatgtatgtgtgtgtgtatatatgtgtatatatgtatacacacacacacacacacatatatatatatatacacacacacacatatatatatggagagagagagagagacagtgtcttgctctgtcgcccaggctggagtgcagtggtacgatcttggctcattgcaacctccgcctcccaggctcaagcgattctcatgtctcagtctcccaagtagctgggattacaggtgtgcaccaccacaccaggctaaccattccatacattttatacaatcatttttaaaaagaagcatgaaccatttcggttttagagaattaagtttttttaaaaaagagactcttaaaaaaaagtcattatatgaataaaatctgctttgtgttaattccgacaaatcattccatcattgagtctgtcaccaattttttttttttgaaatggagtttcgctcttgttgcccaggctggagtgcaatggtacgatctcggctcactgcaaccgccgcctcccgggttcaagtgattctcctgcctcagcctcccgagtagctgggattacaggcatgcgccaccacgcctggctaattttgtattattagttgagacagggtttctccatgttggtcaggctggtctcgaactcctgacctcaagtgatccgctggccttggcctcccaaagtgctgggattacaggcgtgagccaccgtgcctggcccaattttttttttttaataacttgcacacttaacaatattttttatcttcttgggacaacattcttttctccacaaaaacccaattaaggacgttgtgccagtttactcctacttccttcctgttcactgagcttaaagtgggtataggcgagaatgccaaataatgtacataaaatgccaagggcctgattaatggacagtggatccttaaataaaacatatcctccgaataaagtaatgcagaacttgaagtgtccgaacatgttataggtgacaggtgaagtgttcccaatgatccaataaattgataagttcaccatgaaagctattactccagatagcagcaccataagcaaagcagaaactgaccagggaccaaatattcctccttctccaaacactggctcaaagaagggcacagcaaccagcaacatggcagatgacatcggagcctggtagtacagcagctgcattgagttcacttgtaattcatgctgtttggctcctacccacagcgtgagctggattctggtggagaaggttttctggtagcagaaggtctggatggctatgatcaccggcgtggtcatggccttggccagctgataggtgcctatggtgttgttctgcagagaaaggttagtgaagaccacaaagccacagaagctgagggccaggaggaggagcctggagggcggcagacttttgggggcaaagatgtccagcttctggcagatatacaagcccagccaggtgaccacgaagtgcaccagggtcaggctcatgttggggaagccgtggtacacataaatccatttgttgaggaacacaatgcagatggacaccagcaggttgaacaggagcccggcggcgattcgccagtggccccgcactcggtccaccagcaatgccatgatccccgcgaagctggggccgtctagcctcggaaggggcgccgggcctgtctccggctgcccttctactccaccgccgcgtcctcgcagacgccgacctcaccgtctgacccaggagtggcatgcacagatcaaccccgggcgagtagcactcttaacagaggacacacaccccgccgccgccctgtaagccagctaggac

SEQ ID NO: 15655 - RNA, 1917 nt, Homo sapiens
  source 1..1917: mol_type = other RNA
gctgggattacaggcatgagccactgtgcccaggaacttactcttgcctgtaaaaatacagctctgaagtgaagaaatcccaggcgccacatcaaggaggcgaaactagagtccgcaggaggccagccccgcacgaggagtttcaaacactaaggatcctgacagggaaaagttatatgaagcaagaaaggcaatttaaagcgatagtttatcatatgaatgtttcgttcttaaaaatgaacaagctctatttataatgcccatttagaaatgaatccattaaaaaaaatcagtagatcagcacttattttaattactgagatagagtcacacttgacagaagcaagccctgcggtatatggcatcatcacaccaccggtgggtattttaatcctaaaactgagacagagtttacttaaacatttaaggcttgagtttcctctgtacagtgtggaggtgattaagaaaattaatcctaacatgaagatttttcatccagttaaaaaaagaaatactttaaaaacgacctgcccttccaaaacatgaagttaacttggagtttttctgtgatatgacaaactaggcataatcctatctcggaattgttgagtagaaaatttatgtactaatactcctgttaaaattcaacagctttattgtgaaagaatccagagatctcacactgaaaaaatactaacacagctcatatataaattacttatctataagaacaattatagaaggaatctaaatggggcaattttaacaaaccaggcaaaatatcacatatacctgaatataaggtaactccaagccatgagtataagattaaggcagttactttattttgaacaaggaagtggcataagcaactcagtgtgtgccccttagggtgggagctcttccccctaccactccccaccccaaggcatcattttggagaaaaaagtgtcttctatctggctagctgtgttatctaggattgcaccttcttacacggcaggcgcggcatcacgtccagatgggcatctaaggaactgcatttcgggagatgaaactttcatttgggactcaactgaatgcatgaactaacacagggccatggacccaccagtcttgattgagttacagaaaatgaaggtgactctttacacttccaagttgctttctagatcctttcattacaaaatattctgatcaaataatcttacaaaggaaagataatctagcctcaaggctatcctctaaaagcaaagagaaagtgattgattttctgctcagtcattacattggggacctttacgaggcacgtgttagttcccaggcagcactgctaggcggtctgtgccagaaatttcacgtactgcccgcgggcttcaaaatggtcagcgggccggttgtacgctgtccacaccggttctcccacaaacagccgcatggccttcgtgtagttcttctcgtccaccgtgaagcggtgatagatccccgcggggagcgtcaccatgtctcccttctccatgaagatccggatccactggtcctccttgtccctcacatcgaagtacccactgccatccaggatgtagcggatctcatcgtccaagtgcaaatgctcctcgtagaacatcttaatcttttcttcataatttggtagtttatctttgcatatggttatgatgtccatccaggagtagttcctctctcttcggatcttttctaattctggatcattctcatatttgtcagcatccagcttccagtagagcaccccgagccgccgcagctgctccaggcccactgggcggccggggtcggggcggtggggttgccgcgggtcgcccggggcgtcgtccatataccaggcctgcaccatgacgcgcagtgcgggtgccgtgttcgaacccaggggccgcgctc

SEQ ID NO: 15656 - RNA, 4693 nt, Homo sapiens
  source 1..4693: mol_type = other RNA
gctgggattacaggcatgagccactgtgcccaggaacttactcttgcctgtaaaaatacagctctgaagtgaagaaatcccaggcgccacatcaaggaggcgaaactagagtccgcaggaggccagccccgcacgaggagtttcaaacactaaggatcctgacagggaaaagttatatgaagcaagaaaggcaatttaaagcgatagtttatcatatgaatgtttcgttcttaaaaatgaacaagctctatttataatgcccatttagaaatgaatccattaaaaaaaatcagtagatcagcacttattttaattactgagatagagtcacacttgacagaagcaagccctgcggtatatggcatcatcacaccaccggtgggtattttaatcctaaaactgagacagagtttacttaaacatttaaggcttgagtttcctctgtacagtgtggaggtgattaagaaaattaatcctaacatgaagatttttcatccagttaaaaaaagaaatactttaaaaacgacctgcccttccaaaacatgaagttaacttggagtttttctgtgatatgacaaactaggcataatcctatctcggaattgttgagtagaaaatttatgtactaatactcctgttaaaattcaacagctttattgtgaaagaatccagagatctcacactgaaaaaatactaacacagctcatatataaattacttatctataagaacaattatagaaggaatctaaatggggcaattttaacaaaccaggcaaaatatcacatatacctgaatataaggtaactccaagccatgagtataagattaaggcagttactttattttgaacaaggaagtggcataagcaactcagtgtgtgccccttagggtgggagctcttccccctaccactccccaccccaaggcatcattttggagaaaaaagtgtcttctatctggctagctgtgttatctaggattgcaccttcttacacggcaggcgcggcatcacgtccagatgggcatctaaggaactgcatttcgggagatgaaactttcatttgggactcaactgaatgcatgaactaacacagggccatggacccaccagtcttgattgagttacagaaaatgaaggtgactctttacacttccaagttgctttctagatcctttcattacaaaatattctgatcaaataatcttacaaaggaaagataatctagcctcaaggctatcctctaaaagcaaagagaaagtgattgattttctgctcagtcattacattggggacctttacgaggcacgtgttagttcccaggcagcactgctaggcggtctgtgccagaaatttcacgtactgcccgcgggcttcaaaatggtcagcgggccggttgtacgctgtccacaccggttctcccacaaacagccgcatggccttcgtgtagttcttctcgtccaccgtgaagcggtgatagatccccgcggggagcgtcaccatgtctcccttctccatgaagatccggatccactggtcctccttgtccctcacatcgaagtacccactgccatccaggatgtagcggatctcatcgtccaagtgcaaatgctcctcgtagaacatcttaatcttttcttcataatttggtagtttatctttgcatatggttatgatgtccatccaggagtagttcctctctcttcggatcttttctaattctggatcattctcatatttgtcagcatccagtgaacaacaaactccagtgttgcaggaagtcagggaccccgaatggagggaccggctggagccatggcagaggaacataagttttgaagatttcacggacatctatcagttctcaaataatacttttataatttattatgcctgtctttaatctcttaatcctgttatcttcgtaagctgaggatgtatgtcacctcaggaccactgtgataattgtgttaactgtacaaattgattgtaaaacatgtgtgtttgaacaatatgaaatcagtacaccttaaaaaataaaataacagcgatttttagggaacaagggaagacaaccataaggtttgactgcctgcagggtcaggcaaaaacacccatatttttcttcttgcagagagcctataaatgggcgtgcaagtagagaaggtatcactaaattcttttcctaggaaggaatattaatattaatactctggggaaggaatgcatttctggggggaggtctataaacagctgctctgggaatgtctgtcttatgcggttgagataaggactgagatacgccctggtcttctgcagtaccctcaggcttactaaggtggggaaaaactccaccctggtaaatttgtggtcagaccagttctctgctctcgaaccctgttttctgttatttaagatgtttatcaagacaatatgtgcagcactgaacatagatctttatcagtggttctgcttttgccctttgccctgtgatctttgttggacccttatcagtggttctgcttttgccctttgtcctgttccctcagaagcatgtgatctttgttagacccttattagtagttctgctttttgccctttgaagcctgtgatatttgtacctactccctgttcttacaccccctccccttttgaaacccttaataaaaacttgctggtctgagactcaggcgggcatcacggtcctaccgatatgtgatgtcacccctggcggcccagctgtaaaattcctctctttatactgtctctctttatttctcagctggccgacacttatggaaaatggaacctatgttgaaatattgggggtgggttcccccgatactccagaacatattaaagtactagtcatcaatacgttattttctacaaagttgactctaaaacttagcctatccactgcatgatatgcacagtactatttgctatggtctgaatgtgtccatattatgacacataatatgtaatatgacacattatatgacacgtgtcataagtttaaatatacgaatgttgaaacttaacacaaatgtgatagtattaaggggtgggacctttaggatgtgattaagtcatgagggcaagccctcatttataggattagtggccttgtaagagagatggagctgggcactgtggctcacacctataatcccagaactttgggaggccaaggtgggcagatcacctgaggtcaggggttcaagaccagcctgtccaacatggtgaaaccccatctctactaaaaatacaaaaattagccaggcatggtggtccacgcctgtgatcccagctactcgggaggctgaggcaggagaatcacttgaatccaggaggcagaggttgcagtgagccaagactgcgctaccagcctgggtgacagagcgaggctccatctcaaaaaaaaaaaaaaaaaaaaaaaagagcaagagagatgtaagagagcagtttgccccttccaccacatgaggacagagcaaggaaatggccgtctatgaggacaggatcctcatcagacactaaatctgctggcaccttaatcttggacttcttagcctctagaactataagaattctataaattgctgttgtttataaattgcccagtttaagctatttttgtcattttgttatagcagcaggtatttagtttattccaagctaaaataatcttccaattgtttgtatgtatgacaaaaggttttttagaactctatgtcactaataacagattgattaaacagatacacaaacatgtccacatgtgttacctctgttaaaaattatgggagatgttacatatatataatgttaatatggggtgtgtgtgtggcttttttgttttttgggtttttttagagatgaggtctcaaacttctggcttcaggcaatctgccgcctcagcctcccaaagtgctgggatgacagaagccaccatgcctggcccaggagaggtcactgttttggactgagcccctgcactaggccccaggatgagaccaaaccaaaatgcagccactcatgccatatgccacttgatcaaactaaaactttaaagaaggaggtgcatctcaaacagaccagcttttcctgcgatcagaagattccagtcttcctgagtcagaataataaggaagtcgcttctgctttaacccttaggaaaaaagtaacctaatgtaacttgacgttaaccaatcagcttttctacctattgttctgtttctttgttgccgccctacaaaacccactgttgtgctattaccctatcgagctcttattctattttgtagaacggaggttgccctattcacaaatcaagaataaaagctaattagatctttaactaaatttgttgtaattttgtcttccaacagcactgatccagaatggatattaagaaagcatataggccgggtgcggtggttcgtgtctataatgccagcactttgggaggccgaagtgggtggatcacctgaggtcagcagttcaagatcagcctgaccaacatggagaaaccctgtctctactaaaaatacaaaattagcccggcatggtgctgtgcaccttgtaatcccagctactcgggaggctgacacatgagaatggcttgaactcgggaagatgaggttgcggtgagccgagatcatgccactgcactccagcctgggcaaa

SEQ ID NO: 15657 - RNA, 4153 nt, Homo sapiens
  source 1..4153: mol_type = other RNA
gctgggattacaggcatgagccactgtgcccaggccatggtgggtatttttaatggacaagaacccagaatgaagatctacagaggcttcctggaggtggtgggactgaggtcatctggtttggcaggatggaaggccagctttcccagggtggaaccatcagagtggaggccccgcccagaaccaacagcagcaccatgcgcacccatagaaggggtagcctggagggaggccaggcgtgcgcagaaggcagctggacatgtggctacacctcaggttctttcatagacaagttactgacacattgctggctccaggggaaaacgcaaaacgaggaaaaggcccctctccctgctctcagggatgctgtagtcttttgactctcggctgtgccagagcttccccggaagctcctgggaccagcatgcctcccactcaagccagtcagccagcatcttgctcctgggacaggctttgggccatgggagccaggcagaggccccagactagccaaggcccgggctggtcccacctcccgctcctgctcgctcccgacggctgcctaggctggggggctgcagactgtgccctgccgcgcagggactggagatgtggcagccccgccaagggatctcccaagagtcaaaggaggtaatggaggaagaaggatctgaagacgcagggaagtgcccaggcccccgcagggaggctgaaagcagcggtgcctgccacgcccgagaagcaggctccaactcacgtgctcgtcagcagccgcactgctgcctgctttgtcattttatgcttatgtaaaaaaatactttttgcaagaaaaatctacaggtacaaaatgtcatcccagccccatacagtaccaagtaatatataggcatatatatatatatatatatatttatgtatttataacagaaaattggatagaaattattccaggcatatgggatgtggttcccctgggccagaaccacgtagggcagaggagccctgccctccaagtgtgcatgcccaccaaagggacaggggctttcaggagtcacaccagatcacgcttgggacctttttagagcctggctgagccaccctttccagagttccagtgagcagggggcccctcagtgcatcttccccacctcccctgcttccagggacgctgggctgcagacttcgcagctgctgccacatggggttggagcctccaacagcatcatccctgagtagacctggtccactgagtcccacaggtcggctctctgcagcctttccctgcaggtcaccaccctctacaggcaatggcaaggacgcgacatcacaggtagacagcccacatcctctcatccttccggtctcctggactggagttgtcccggtgccctggagacccagtcactgccacctctcccctgcctggactcagcaggggaaagactggaggccctgctcctgccctttggctctgccagcacccccgaccagccctatatctcctcctccaccttcaagatcatccctgagaagacctcgagccccgagtgggtgcccttggggctgtcctgggagcctccagcaggcccctgggccactccactggcaggactaccgtcctggagtgagggtgaggcttcccgggtagggcgtgcttccaccagcctctcgagggtccggttgagggcctccacgccatcggccagacgctggctctgctcggccagccgctgcagcagcaggttttgctgggccatgagtgtgctctgctgctgggcccaggaggacagcagggcgccctgctgccggtgggagtccagcagctgctgctcaaatgcggacgtttcagatgctgccgctggggtcctcctggagggcaagggaggtgctggcgccgaagagggcggggaaggctggaaggcccccatgagtgtggttgctggtggggtggaggctggggaagcaggtggggagggtgaggaggtgggtgcgtggaagactcctcgtaagtccagggggtcaggttcaggcaggctgggcccttccagggacctcaggggcagccacaagcagctgggggtctcgtcctcctcatcagttggcaggggctccgtggtctggccctcgccttggggaccgtgggcagaaaaggtctctgccaccatgcgctccacaggtgtgaggaggaggccgggggcggggccgccctccgccagcttcttgcgcacagcacctcgcaggtcccgccacttgtgcttgaggtcccccaggtcgcggcggcagtagcccagcgcgttcactgcctgcaggatgcggctccacacgcggtgctttcgggcaggtgtgccccgcagcgccccgaacagcagcgggtagtggcgccgcaccctctgcaccagcacctccgtctcctgggggctgaagttgggcttgcgtgtcttggtgcgggagtgggggcccggccgcaggggtgtggagcccggcccggcacccagcagcagggctgccgcggccggctcggggctgcagctctgctggcagatggctttgctgctgctggacccaacagcttctccttgctctgacaccatggaggccaagtccttgatgatctgattcacatccagcaagttgctctccatctgcaggatggcctcctcccgcagccggatggcctccaggtcctcttcagtgatgtccgggagcagcgcctgctcctggccctgccacatgttgtcactcccgttaaagaccttctcatcatcagccagctcggcaaacggggcctggggactctgctgtttactgcccctctgcgccatgggaagcagcgctctggacttttctgcaattttcttctgcaccactccatagcactgaatggcatctgagagctgggttttcagccggtccagctgaggacgctcctgctgcagacgctccgggcaggagctgcgcagcagctcggccatctgcttcacggagctggcgctggctgcaatggtcttgttggtctcctgctgtgccgtgtgcaggctgtcccgaagctcctgcgtgtcactcggtgtccctaaggactgaaggctccgctccaaggaggtcacactggagttgattcggaagacgttggccgacatctcctggaacagctcctggaggttgcacggatcgacctgggtggctctgggcggctccagactgaagccctcggagggcagggcctggcaagagaaggtcttggccaccacctgctccacgggcgtgagagccagggcctggggcttgccggaaccagggctggggccatgggccgccttccggaggtcgcccagcttgcgccgcacgacggctcgtaggtcccgccacttgtgcttcaggtccacaacgtcgcggcgacagtagcccagcgcattcacggcctgcaggatgcggctccacacgcggtacctgcgagtgggctcggccttcagcagccccgtgccaaacagcagctggtggtgcttgctcaccttggacaccagcacctcggtctcctgcgggcagaagttgggcttcctcttcttggcccgggtagtgctgggccccgccatccggccatggggcccagcagccgagtccttcctcgggccaatggtgggtgatgaggtgggctccggcatccggctgccttcaggggcaaccccaggccctcgcttcctggcccttgggacaataggcgtgcctgctggccccagatcaccttccccgtccttccccacacagcggttctgcagcttgctctctggcgacgggcaggggaaatggcggattccatactcggtccaacatctagcgcactctaggggctgacagccttgtctcgaaggtcccccgaaagggccacggctccccaggccacctccacgggcgatggatccgtatgacatcttcttacagatggcagggccagcagcctccacactgagctgggcctcggtggctcgcggaccgctccgggcgctcacggcgggcgaggcgggcggggcgggcacccaaacatcacgtgacggcccctcccgccgccggcgtgcgcgccccctcccgcaccagccaatggccgccggtcccggacgcgcgcggggactacccgccccagaggccccggcgcggagcc

SEQ ID NO: 15658 - RNA, 3311 nt, Homo sapiens
  source 1..3311: mol_type = other RNA
gctgggattacaggcatgagccactgtgcccaggccatggtgggtatttttaatggacaagaacccagaatgaagatctacagaggcttcctggaggtggtgggactgaggtcatctggtttggcaggatggaaggccagctttcccagggtggaaccatcagagtggaggccccgcccagaaccaacagcagcaccatgcgcacccatagaaggggtagcctggagggaggccaggcgtgcgcagaaggcagctggacatgtggctacacctcaggttctttcatagacaagttactgacacattgctggctccaggggaaaacgcaaaacgaggaaaaggcccctctccctgctctcagggatgctgtagtcttttgactctcggctgtgccagagcttccccggaagctcctgggaccagcatgcctcccactcaagccagtcagccagcatcttgctcctgggacaggctttgggccatgggagccaggcagaggccccagactagccaaggcccgggctggtcccacctcccgctcctgctcgctcccgacggctgcctaggctggggggctgcagactgtgccctgccgcgcagggactggagatgtggcagccccgccaagggatctcccaagagtcaaaggaggtaatggaggaagaaggatctgaagacgcagggaagtgcccaggcccccgcagggaggctgaaagcagcggtgcctgccacgcccgagaagcaggctccaactcacgtgctcgtcagcagccgcactgctgcctgctttgtcattttatgcttatgtaaaaaaatactttttgcaagaaaaatctacaggtacaaaatgtcatcccagccccatacagtaccaagtaatatataggcatatatatatatatatatatatttatgtatttataacagaaaattggatagaaattattccaggcatatgggatgtggttcccctgggccagaaccacgtagggcagaggagccctgccctccaagtgtgcatgcccaccaaagggacaggggctttcaggagtcacaccagatcacgcttgggacctttttagagcctggctgagccaccctttccagagttccagtgagcagggggcccctcagtgcatcttccccacctcccctgcttccagggacgctgggctgcagacttcgcagctgctgccacatggggttggagcctccaacagcatcatccctgagtagacctggtccactgagtcccacaggtcggctctctgcagcctttccctgcaggtcaccaccctctacaggcaatggcaaggacgcgacatcacaggtagacagcccacatcctctcatccttccggtctcctggactggagttgtcccggtgccctggagacccagtcactgccacctctcccctgcctggactcagcaggggaaagactggaggccctgctcctgccctttggctctgccagcacccccgaccagccctatatctcctcctccaccttcaagatcatccctgagaagacctcgagccccgagtgggtgcccttggggctgtcctgggagcctccagcaggcccctgggccactccactggcaggactaccgtcctggagtgagggtgaggcttcccgggtagggcgtgcttccaccagcctctcgagggtccggttgagggcctccacgccatcggccagacgctggctctgctcggccagccgctgcagcagcaggttttgctgggccatgagtgtgctctgctgctgggcccaggaggacagcagggcgccctgctgccggtgggagtccagcagctgctgctcaaatgcggacgtttcagatgctgccgctggggtcctcctggagggcaagggaggtgctggcgccgaagagggcggggaaggctggaaggcccccatgagtgtggttgctggtggggtggaggctggggaagcaggtggggagggtgaggaggtgggtgcgtggaagactcctcgtaagtccagggggtcaggttcaggcaggctgggcccttccagggacctcaggggcagccacaagcagctgggggtctcgtcctcctcatcagttggcaggggctccgtggtctggccctcgccttggggaccgtgggcagaaaaggtctctgccaccatgcgctccacaggtgtgaggaggaggccgggggcggggccgccctccgccagcttcttgcgcacagcacctcgcaggtcccgccacttgtgcttgaggtcccccaggtcgcggcggcagtagcccagcgcgttcactgcctgcaggatgcggctccacacgcggtgctttcgggcaggtgtgccccgcagcgccccgaacagcagcgggtagtggcgccgcaccctctgcaccagcacctccgtctcctgggggctgaagttgggcttgcgtgtcttggtgcgggagtgggggcccggccgcaggggtgtggagcccggcccggcacccagcagcagggctgccgcggccggctcggggctgcagctctgctggcagatggctttgctgctgctggacccaacagcttctccttgctctgacaccatggaggccaagtccttgatgatctgattcacatccagcaagttgctctccatctgcaggatggcctcctcccgcagccggatggcctccaggtcctcttcagtgatgtccgggagcagcgcctgctcctggccctgccacatgttgtcactcccgttaaagaccttctcatcatcagccagctcggcaaacggggcctggggactctgctgtttactgcccctctgcgccatgggaagcagcgctctggacttttctgcaattttcttctgcaccactccatagcactgaatggcatctgagagctgggttttcagccggtccagctgaggacgctcctgctgcagacgctcctgcgggcaggagctgcgcagcagctcggccatctgcttcacggagctggcgctggctgcaatggtcttgttggtctcctgctgtgccgtgtgcaggctgtcccgaagctcctgcgtgtcactcggtgtccctaaggactgaaggctccgctccaaggaggtcacactggagttgattcggaagacgttggccgacatctcctggaacagctcctggaggttgcacggatcgacctgggtggctaggggctgacagccttgtctcgaaggtcccccgaaagggccacggctccccaggccacctccacgggcgatggatccgtatgacatcttcttacagatggcagggccagcagcctccacactgag

SEQ ID NO: 15659 - RNA, 3818 nt, Homo sapiens
  source 1..3818: mol_type = other RNA
gctgggattacaggcatgagccactgtgcccaggccatggtgggtatttttaatggacaagaacccagaatgaagatctacagaggcttcctggaggtggtgggactgaggtcatctggtttggcaggatggaaggccagctttcccagggtggaaccatcagagtggaggccccgcccagaaccaacagcagcaccatgcgcacccatagaaggggtagcctggagggaggccaggcgtgcgcagaaggcagctggacatgtggctacacctcaggttctttcatagacaagttactgacacattgctggctccaggggaaaacgcaaaacgaggaaaaggcccctctccctgctctcagggatgctgtagtcttttgactctcggctgtgccagagcttccccggaagctcctgggaccagcatgcctcccactcaagccagtcagccagcatcttgctcctgggacaggctttgggccatgggagccaggcagaggccccagactagccaaggcccgggctggtcccacctcccgctcctgctcgctcccgacggctgcctaggctggggggctgcagactgtgccctgccgcgcagggactggagatgtggcagccccgccaagggatctcccaagagtcaaaggaggtaatggaggaagaaggatctgaagacgcagggaagtgcccaggcccccgcagggaggctgaaagcagcggtgcctgccacgcccgagaagcaggctccaactcacgtgctcgtcagcagccgcactgctgcctgctttgtcattttatgcttatgtaaaaaaatactttttgcaagaaaaatctacaggtacaaaatgtcatcccagccccatacagtaccaagtaatatataggcatatatatatatatatatatatttatgtatttataacagaaaattggatagaaattattccaggcatatgggatgtggttcccctgggccagaaccacgtagggcagaggagccctgccctccaagtgtgcatgcccaccaaagggacaggggctttcaggagtcacaccagatcacgcttgggacctttttagagcctggctgagccaccctttccagagttccagtgagcagggggcccctcagtgcatcttccccacctcccctgcttccagggacgctgggctgcagacttcgcagctgctgccacatggggttggagcctccaacagcatcatccctgagtagacctggtccactgagtcccacaggtcggctctctgcagcctttccctgcaggtcaccaccctctacaggcaatggcaaggacgcgacatcacaggtagacagcccacatcctctcatccttccggtctcctggactggagttgtcccggtgccctggagacccagtcactgccacctctcccctgcctggactcagcaggggaaagactggaggccctgctcctgccctttggctctgccagcacccccgaccagccctatatctcctcctccaccttcaagatcatccctgagaagacctcgagccccgagtgggtgcccttggggctgtcctgggagcctccagcaggcccctgggccactccactggcaggactaccgtcctggagtgagggtgaggcttcccgggtagggcgtgcttccaccagcctctcgagggtccggttgagggcctccacgccatcggccagacgctggctctgctcggccagccgctgcagcagcaggttttgctgggccatgagtgtgctctgctgctgggcccaggaggacagcagggcgccctgctgccggtgggagtccagcagctgctgctcaaatgcggacgtttcagatgctgccgctggggtcctcctggagggcaagggaggtgctggcgccgaagagggcggggaaggctggaaggcccccatgagtgtggttgctggtggggtggaggctggggaagcaggtggggagggtgaggaggtgggtgcgtggaagactcctcgtaagtccagggggtcaggttcaggcaggctgggcccttccagggacctcaggggcagccacaagcagctgggggtctcgtcctcctcatcagttggcaggggctccgtggtctggccctcgccttggggaccgtgggcagaaaaggtctctgccaccatgcgctccacaggtgtgaggaggaggccgggggcggggccgccctccgccagcttcttgcgcacagcacctcgcaggtcccgccacttgtgcttgaggtcccccaggtcgcggcggcagtagcccagcgcgttcactgcctgcaggatgcggctccacacgcggtgctttcgggcaggtgtgccccgcagcgccccgaacagcagcgggtagtggcgccgcaccctctgcaccagcacctccgtctcctgggggctgaagttgggcttgcgtgtcttggtgcgggagtgggggcccggccgcaggggtgtggagcccggcccggcacccagcagcagggctgccgcggccggctcggggctgcagctctgctggcagatggctttgctgctgctggacccaacagcttctccttgctctgacaccatggaggccaagtccttgatgatctgattcacatccagcaagttgctctccatctgcaggatggcctcctcccgcagccggatggcctccaggtcctcttcagtgatgtccgggagcagcgcctgctcctggccctgccacatgttgtcactcccgttaaagaccttctcatcatcagccagctcggcaaacggggcctggggactctgctgtttactgcccctctgcgccatgggaagcagcgctctggacttttctgcaattttcttctgcaccactccatagcactgaatggcatctgagagctgggttttcagccggtccagctgaggacgctcctgctgcagacgctcctgcgggcaggagctgcgcagcagctcggccatctgcttcacggagctggcgctggctgcaatggtcttgttggtctcctgctgtgccgtgtgcaggctgtcccgaagctcctgcgtgtcactcggtgtccctaaggactgaaggctccgctccaaggaggtcacactggagttgattcggaagacgttggccgacatctcctggaacagctcctggaggttgcacggatcgacctgggtggctctgggcggctccagactgaagccctcggagggcagggcctggcaagagaaggtcttggccaccacctgctccacgggcgtgagagccagggcctggggcttgccggaaccagggctggggccatgggccgccttccggaggtcgcccagcttgcgccgcacgacggctcgtaggtcccgccacttgtgcttcaggtccacaacgtcgcggcgacagtagcccagcgcattcacggcctgcaggatgcggctccacacgcggtacctgcgagtgggctcggccttcagcagccccgtgccaaacagcagctggtggtgcttgctcaccttggacaccagcacctcggtctcctgcgggcagaagttgggcttcctcttcttggcccgggtagtgctgggccccgccatccggccatggggcccagcagccgagtccttcctcgggccaatggtgggtgatgaggtgggctccggcatccggctgccttcaggggcaaccccaggccctaggggctgacagccttgtctcgaaggtcccccgaaagggccacggctccccaggccacctccacgggcgatggatccgtatgacatcttcttacagatggcagggccagcagcctccacactgag

SEQ ID NO: 15660 - RNA, 4153 nt, Homo sapiens
  source 1..4153: mol_type = other RNA
gctgggattacaggcatgagccactgtgcccaggccatggtgggtatttttaatggacaagaacccagaatgaagatctacagaggcttcctggaggtggtgggactgaggtcatctggtttggcaggatggaaggccagctttcccagggtggaaccatcagagtggaggccccgcccagaaccaacagcagcaccatgcgcacccatagaaggggtagcctggagggaggccaggcgtgcgcagaaggcagctggacatgtggctacacctcaggttctttcatagacaagttactgacacattgctggctccaggggaaaacgcaaaacgaggaaaaggcccctctccctgctctcagggatgctgtagtcttttgactctcggctgtgccagagcttccccggaagctcctgggaccagcatgcctcccactcaagccagtcagccagcatcttgctcctgggacaggctttgggccatgggagccaggcagaggccccagactagccaaggcccgggctggtcccacctcccgctcctgctcgctcccgacggctgcctaggctggggggctgcagactgtgccctgccgcgcagggactggagatgtggcagccccgccaagggatctcccaagagtcaaaggaggtaatggaggaagaaggatctgaagacgcagggaagtgcccaggcccccgcagggaggctgaaagcagcggtgcctgccacgcccgagaagcaggctccaactcacgtgctcgtcagcagccgcactgctgcctgctttgtcattttatgcttatgtaaaaaaatactttttgcaagaaaaatctacaggtacaaaatgtcatcccagccccatacagtaccaagtaatatataggcatatatatatatatatatatatttatgtatttataacagaaaattggatagaaattattccaggcatatgggatgtggttcccctgggccagaaccacgtagggcagaggagccctgccctccaagtgtgcatgcccaccaaagggacaggggctttcaggagtcacaccagatcacgcttgggacctttttagagcctggctgagccaccctttccagagttccagtgagcagggggcccctcagtgcatcttccccacctcccctgcttccagggacgctgggctgcagacttcgcagctgctgccacatggggttggagcctccaacagcatcatccctgagtagacctggtccactgagtcccacaggtcggctctctgcagcctttccctgcaggtcaccaccctctacaggcaatggcaaggacgcgacatcacaggtagacagcccacatcctctcatccttccggtctcctggactggagttgtcccggtgccctggagacccagtcactgccacctctcccctgcctggactcagcaggggaaagactggaggccctgctcctgccctttggctctgccagcacccccgaccagccctatatctcctcctccaccttcaagatcatccctgagaagacctcgagccccgagtgggtgcccttggggctgtcctgggagcctccagcaggcccctgggccactccactggcaggactaccgtcctggagtgagggtgaggcttcccgggtagggcgtgcttccaccagcctctcgagggtccggttgagggcctccacgccatcggccagacgctggctctgctcggccagccgctgcagcagcaggttttgctgggccatgagtgtgctctgctgctgggcccaggaggacagcagggcgccctgctgccggtgggagtccagcagctgctgctcaaatgcggacgtttcagatgctgccgctggggtcctcctggagggcaagggaggtgctggcgccgaagagggcggggaaggctggaaggcccccatgagtgtggttgctggtggggtggaggctggggaagcaggtggggagggtgaggaggtgggtgcgtggaagactcctcgtaagtccagggggtcaggttcaggcaggctgggcccttccagggacctcaggggcagccacaagcagctgggggtctcgtcctcctcatcagttggcaggggctccgtggtctggccctcgccttggggaccgtgggcagaaaaggtctctgccaccatgcgctccacaggtgtgaggaggaggccgggggcggggccgccctccgccagcttcttgcgcacagcacctcgcaggtcccgccacttgtgcttgaggtcccccaggtcgcggcggcagtagcccagcgcgttcactgcctgcaggatgcggctccacacgcggtgctttcgggcaggtgtgccccgcagcgccccgaacagcagcgggtagtggcgccgcaccctctgcaccagcacctccgtctcctgggggctgaagttgggcttgcgtgtcttggtgcgggagtgggggcccggccgcaggggtgtggagcccggcccggcacccagcagcagggctgccgcggccggctcggggctgcagctctgctggcagatggctttgctgctgctggacccaacagcttctccttgctctgacaccatggaggccaagtccttgatgatctgattcacatccagcaagttgctctccatctgcaggatggcctcctcccgcagccggatggcctccaggtcctcttcagtgatgtccgggagcagcgcctgctcctggccctgccacatgttgtcactcccgttaaagaccttctcatcatcagccagctcggcaaacggggcctggggactctgctgtttactgcccctctgcgccatgggaagcagcgctctggacttttctgcaattttcttctgcaccactccatagcactgaatggcatctgagagctgggttttcagccggtccagctgaggacgctcctgctgcagacgctcctgcgggcaggagctgcgcagcagctcggccatctgcttcacggagctggcgctggctgcaatggtcttgttggtctcctgctgtgccgtgtgcaggctgtcccgaagctcctgcgtgtcactcggtgtccctaaggactgaaggctccgctccaaggaggtcacactggagttgattcggaagacgttggccgacatctcctggaacagctcctggaggttgcacggatcgacctgggtggctctgggcggctccagactgaagccctcggagggcagggcctggcaagagaaggtcttggccaccacctgctccacgggcgtgagagccagggcctggggcttgccggaaccagggctggggccatgggccgccttccggaggtcgcccagcttgcgccgcacgacggctcgtaggtcccgccacttgtgcttcaggtccacaacgtcgcggcgacagtagcccagcgcattcacggcctgcaggatgcggctccacacgcggtacctgcgagtgggctcggccttcagcagccccgtgccaaacagcagctggtggtgcttgctcaccttggacaccagcacctcggtctcctgcgggcagaagttgggcttcctcttcttggcccgggtagtgctgggccccgccatccggccatggggcccagcagccgagtccttcctcgggccaatggtgggtgatgaggtgggctccggcatccggctgccttcaggggcaaccccaggccctcgcttcctggcccttgggacaataggcgtgcctgctggccccagatcaccttccccgtccttccccacacagcggttctgcagcttgctctctggcgacgggcaggggaaatggcggattccatactcggtccaacatctagcgcactctaggggctgacagccttgtctcgaaggtcccccgaaagggccacggctccccaggccacctccacgggcgatggatccgtatgacatcttcttacagatggcagggccagcagcctccacactgagcatgttcatggacaggaacactcaagactgtgcagctacagcagctgatggttttgtagaggaatttggctgaacatttccaatgtgccaaaaattgtcccaggacactgggcctcggtggctcgcggaccgctccgggcgctcacggcgggcgaggcgggcggggcgggcacccaaacatcacg

SEQ ID NO: 15661 - RNA, 3993 nt, Homo sapiens
  source 1..3993: mol_type = other RNA
gctgggattacaggcatgagccactgtgcccaggccatggtgggtatttttaatggacaagaacccagaatgaagatctacagaggcttcctggaggtggtgggactgaggtcatctggtttggcaggatggaaggccagctttcccagggtggaaccatcagagtggaggccccgcccagaaccaacagcagcaccatgcgcacccatagaaggggtagcctggagggaggccaggcgtgcgcagaaggcagctggacatgtggctacacctcaggttctttcatagacaagttactgacacattgctggctccaggggaaaacgcaaaacgaggaaaaggcccctctccctgctctcagggatgctgtagtcttttgactctcggctgtgccagagcttccccggaagctcctgggaccagcatgcctcccactcaagccagtcagccagcatcttgctcctgggacaggctttgggccatgggagccaggcagaggccccagactagccaaggcccgggctggtcccacctcccgctcctgctcgctcccgacggctgcctaggctggggggctgcagactgtgccctgccgcgcagggactggagatgtggcagccccgccaagggatctcccaagagtcaaaggaggtaatggaggaagaaggatctgaagacgcagggaagtgcccaggcccccgcagggaggctgaaagcagcggtgcctgccacgcccgagaagcaggctccaactcacgtgctcgtcagcagccgcactgctgcctgctttgtcattttatgcttatgtaaaaaaatactttttgcaagaaaaatctacaggtacaaaatgtcatcccagccccatacagtaccaagtaatatataggcatatatatatatatatatatatttatgtatttataacagaaaattggatagaaattattccaggcatatgggatgtggttcccctgggccagaaccacgtagggcagaggagccctgccctccaagtgtgcatgcccaccaaagggacaggggctttcaggagtcacaccagatcacgcttgggacctttttagagcctggctgagccaccctttccagagttccagtgagcagggggcccctcagtgcatcttccccacctcccctgcttccagggacgctgggctgcagacttcgcagctgctgccacatggggttggagcctccaacagcatcatccctgagtagacctggtccactgagtcccacaggtcggctctctgcagcctttccctgcaggtcaccaccctctacaggcaatggcaaggacgcgacatcacaggtagacagcccacatcctctcatccttccggtctcctggactggagttgtcccggtgccctggagacccagtcactgccacctctcccctgcctggactcagcaggggaaagactggaggccctgctcctgccctttggctctgccagcacccccgaccagccctatatctcctcctccaccttcaagatcatccctgagaagacctcgagccccgagtgggtgcccttggggctgtcctgggagcctccagcaggcccctgggccactccactggcaggactaccgtcctggagtgagggtgaggcttcccgggtagggcgtgcttccaccagcctctcgagggtccggttgagggcctccacgccatcggccagacgctggctctgctcggccagccgctgcagcagcaggttttgctgggccatgagtgtgctctgctgctgggcccaggaggacagcagggcgccctgctgccggtgggagtccagcagctgctgctcaaatgcggacgtttcagatgctgccgctggggtcctcctggagggcaagggaggtgctggcgccgaagagggcggggaaggctggaaggcccccatgagtgtggttgctggtggggtggaggctggggaagcaggtggggagggtgaggaggtgggtgcgtggaagactcctcgtaagtccagggggtcaggttcaggcaggctgggcccttccagggacctcaggggcagccacaagcagctgggggtctcgtcctcctcatcagttggcaggggctccgtggtctggccctcgccttggggaccgtgggcagaaaaggtctctgccaccatgcgctccacaggtgtgaggaggaggccgggggcggggccgccctccgccagcttcttgcgcacagcacctcgcaggtcccgccacttgtgcttgaggtcccccaggtcgcggcggcagtagcccagcgcgttcactgcctgcaggatgcggctccacacgcggtgctttcgggcaggtgtgccccgcagcgccccgaacagcagcgggtagtggcgccgcaccctctgcaccagcacctccgtctcctgggggctgaagttgggcttgcgtgtcttggtgcgggagtgggggcccggccgcaggggtgtggagcccggcccggcacccagcagcagggctgccgcggccggctcggggctgcagctctgctggcagatggctttgctgctgctggacccaacagcttctccttgctctgacaccatggaggccaagtccttgatgatctgattcacatccagcaagttgctctccatctgcaggatggcctcctcccgcagccggatggcctccaggtcctcttcagtgatgtccgggagcagcgcctgctcctggccctgccacatgttgtcactcccgttaaagaccttctcatcatcagccagctcggcaaacggggcctggggactctgctgtttactgcccctctgcgccatgggaagcagcgctctggacttttctgcaattttcttctgcaccactccatagcactgaatggcatctgagagctgggttttcagccggtccagctgaggacgctcctgctgcagacgctcctgcgggcaggagctgcgcagcagctcggccatctgcttcacggagctggcgctggctgcaatggtcttgttggtctcctgctgtgccgtgtgcaggctgtcccgaagctcctgcgtgtcactcggtgtccctaaggactgaaggctccgctccaaggaggtcacactggagttgattcggaagacgttggccgacatctcctggaacagctcctggaggttgcacggatcgacctgggtggctctgggcggctccagactgaagccctcggagggcagggcctggcaagagaaggtcttggccaccacctgctccacgggcgtgagagccagggcctggggcttgccggaaccagggctggggccatgggccgccttccggaggtcgcccagcttgcgccgcacgacggctcgtaggtcccgccacttgtgcttcaggtccacaacgtcgcggcgacagtagcccagcgcattcacggcctgcaggatgcggctccacacgcggtacctgcgagtgggctcggccttcagcagccccgtgccaaacagcagctggtggtgcttgctcaccttggacaccagcacctcggtctcctgcgggcagaagttgggcttcctcttcttggcccgggtagtgctgggccccgccatccggccatggggcccagcagccgagtccttcctcgggccaatggtgggtgatgaggtgggctccggcatccggctgccttcaggggcaaccccaggccctcgcttcctggcccttgggacaataggcgtgcctgctggccccagatcaccttccccgtccttccccacacagcggttctgcagcttgctctctggcgacgggcaggggaaatggcggattccatactcggtccaacatctagcgcactctaggggctgacagccttgtctcgaaggtcccccgaaagggccacggctccccaggccacctccacgggcgatggatccgtatgacatcttcttacagatggcagggccagcagcctccacactgagctccaggcgcaggcaccggctgccc

SEQ ID NO: 15662 - RNA, 4156 nt, Homo sapiens
  source 1..4156: mol_type = other RNA
gctgggattacaggcatgagccactgtgcccaggccatggtgggtatttttaatggacaagaacccagaatgaagatctacagaggcttcctggaggtggtgggactgaggtcatctggtttggcaggatggaaggccagctttcccagggtggaaccatcagagtggaggccccgcccagaaccaacagcagcaccatgcgcacccatagaaggggtagcctggagggaggccaggcgtgcgcagaaggcagctggacatgtggctacacctcaggttctttcatagacaagttactgacacattgctggctccaggggaaaacgcaaaacgaggaaaaggcccctctccctgctctcagggatgctgtagtcttttgactctcggctgtgccagagcttccccggaagctcctgggaccagcatgcctcccactcaagccagtcagccagcatcttgctcctgggacaggctttgggccatgggagccaggcagaggccccagactagccaaggcccgggctggtcccacctcccgctcctgctcgctcccgacggctgcctaggctggggggctgcagactgtgccctgccgcgcagggactggagatgtggcagccccgccaagggatctcccaagagtcaaaggaggtaatggaggaagaaggatctgaagacgcagggaagtgcccaggcccccgcagggaggctgaaagcagcggtgcctgccacgcccgagaagcaggctccaactcacgtgctcgtcagcagccgcactgctgcctgctttgtcattttatgcttatgtaaaaaaatactttttgcaagaaaaatctacaggtacaaaatgtcatcccagccccatacagtaccaagtaatatataggcatatatatatatatatatatatttatgtatttataacagaaaattggatagaaattattccaggcatatgggatgtggttcccctgggccagaaccacgtagggcagaggagccctgccctccaagtgtgcatgcccaccaaagggacaggggctttcaggagtcacaccagatcacgcttgggacctttttagagcctggctgagccaccctttccagagttccagtgagcagggggcccctcagtgcatcttccccacctcccctgcttccagggacgctgggctgcagacttcgcagctgctgccacatggggttggagcctccaacagcatcatccctgagtagacctggtccactgagtcccacaggtcggctctctgcagcctttccctgcaggtcaccaccctctacaggcaatggcaaggacgcgacatcacaggtagacagcccacatcctctcatccttccggtctcctggactggagttgtcccggtgccctggagacccagtcactgccacctctcccctgcctggactcagcaggggaaagactggaggccctgctcctgccctttggctctgccagcacccccgaccagccctatatctcctcctccaccttcaagatcatccctgagaagacctcgagccccgagtgggtgcccttggggctgtcctgggagcctccagcaggcccctgggccactccactggcaggactaccgtcctggagtgagggtgaggcttcccgggtagggcgtgcttccaccagcctctcgagggtccggttgagggcctccacgccatcggccagacgctggctctgctcggccagccgctgcagcagcaggttttgctgggccatgagtgtgctctgctgctgggcccaggaggacagcagggcgccctgctgccggtgggagtccagcagctgctgctcaaatgcggacgtttcagatgctgccgctggggtcctcctggagggcaagggaggtgctggcgccgaagagggcggggaaggctggaaggcccccatgagtgtggttgctggtggggtggaggctggggaagcaggtggggagggtgaggaggtgggtgcgtggaagactcctcgtaagtccagggggtcaggttcaggcaggctgggcccttccagggacctcaggggcagccacaagcagctgggggtctcgtcctcctcatcagttggcaggggctccgtggtctggccctcgccttggggaccgtgggcagaaaaggtctctgccaccatgcgctccacaggtgtgaggaggaggccgggggcggggccgccctccgccagcttcttgcgcacagcacctcgcaggtcccgccacttgtgcttgaggtcccccaggtcgcggcggcagtagcccagcgcgttcactgcctgcaggatgcggctccacacgcggtgctttcgggcaggtgtgccccgcagcgccccgaacagcagcgggtagtggcgccgcaccctctgcaccagcacctccgtctcctgggggctgaagttgggcttgcgtgtcttggtgcgggagtgggggcccggccgcaggggtgtggagcccggcccggcacccagcagcagggctgccgcggccggctcggggctgcagctctgctggcagatggctttgctgctgctggacccaacagcttctccttgctctgacaccatggaggccaagtccttgatgatctgattcacatccagcaagttgctctccatctgcaggatggcctcctcccgcagccggatggcctccaggtcctcttcagtgatgtccgggagcagcgcctgctcctggccctgccacatgttgtcactcccgttaaagaccttctcatcatcagccagctcggcaaacggggcctggggactctgctgtttactgcccctctgcgccatgggaagcagcgctctggacttttctgcaattttcttctgcaccactccatagcactgaatggcatctgagagctgggttttcagccggtccagctgaggacgctcctgctgcagacgctcctgcgggcaggagctgcgcagcagctcggccatctgcttcacggagctggcgctggctgcaatggtcttgttggtctcctgctgtgccgtgtgcaggctgtcccgaagctcctgcgtgtcactcggtgtccctaaggactgaaggctccgctccaaggaggtcacactggagttgattcggaagacgttggccgacatctcctggaacagctcctggaggttgcacggatcgacctgggtggctctgggcggctccagactgaagccctcggagggcagggcctggcaagagaaggtcttggccaccacctgctccacgggcgtgagagccagggcctggggcttgccggaaccagggctggggccatgggccgccttccggaggtcgcccagcttgcgccgcacgacggctcgtaggtcccgccacttgtgcttcaggtccacaacgtcgcggcgacagtagcccagcgcattcacggcctgcaggatgcggctccacacgcggtacctgcgagtgggctcggccttcagcagccccgtgccaaacagcagctggtggtgcttgctcaccttggacaccagcacctcggtctcctgcgggcagaagttgggcttcctcttcttggcccgggtagtgctgggccccgccatccggccatggggcccagcagccgagtccttcctcgggccaatggtgggtgatgaggtgggctccggcatccggctgccttcaggggcaaccccaggccctcgcttcctggcccttgggacaataggcgtgcctgctggccccagatcaccttccccgtccttccccacacagcggttctgcagcttgctctctggcgacgggcaggggaaatggcggattccatactcggtccaacatctagcgcactctaggggctgacagccttgtctcgaaggtcccccgaaagggccacggctccccaggccacctccacgggcgatggatccgtatgacatcttcttacagatggcagggccagcagcctccacactgagctgggcctcggtggctcgcggaccgctccgggcgctcacggcgggcgaggcgggcggggcgggcacccaaacatcacgtgacggcccctcccgccgccggcgtgcgcgccccctcccgcaccagccaatggccgccggtcccggacgcgcgcggggactacccgccccagaggccccggcgcggagcc

SEQ ID NO: 15663 - RNA, 4067 nt, Homo sapiens
  source 1..4067: mol_type = other RNA
gctgggattacaggcatgagccactgtgcccaggccatggtgggtatttttaatggacaagaacccagaatgaagatctacagaggcttcctggaggtggtgggactgaggtcatctggtttggcaggatggaaggccagctttcccagggtggaaccatcagagtggaggccccgcccagaaccaacagcagcaccatgcgcacccatagaaggggtagcctggagggaggccaggcgtgcgcagaaggcagctggacatgtggctacacctcaggttctttcatagacaagttactgacacattgctggctccaggggaaaacgcaaaacgaggaaaaggcccctctccctgctctcagggatgctgtagtcttttgactctcggctgtgccagagcttccccggaagctcctgggaccagcatgcctcccactcaagccagtcagccagcatcttgctcctgggacaggctttgggccatgggagccaggcagaggccccagactagccaaggcccgggctggtcccacctcccgctcctgctcgctcccgacggctgcctaggctggggggctgcagactgtgccctgccgcgcagggactggagatgtggcagccccgccaagggatctcccaagagtcaaaggaggtaatggaggaagaaggatctgaagacgcagggaagtgcccaggcccccgcagggaggctgaaagcagcggtgcctgccacgcccgagaagcaggctccaactcacgtgctcgtcagcagccgcactgctgcctgctttgtcattttatgcttatgtaaaaaaatactttttgcaagaaaaatctacaggtacaaaatgtcatcccagccccatacagtaccaagtaatatataggcatatatatatatatatatatatttatgtatttataacagaaaattggatagaaattattccaggcatatgggatgtggttcccctgggccagaaccacgtagggcagaggagccctgccctccaagtgtgcatgcccaccaaagggacaggggctttcaggagtcacaccagatcacgcttgggacctttttagagcctggctgagccaccctttccagagttccagtgagcagggggcccctcagtgcatcttccccacctcccctgcttccagggacgctgggctgcagacttcgcagctgctgccacatggggttggagcctccaacagcatcatccctgagtagacctggtccactgagtcccacaggtcggctctctgcagcctttccctgcaggtcaccaccctctacaggcaatggcaaggacgcgacatcacaggtagacagcccacatcctctcatccttccggtctcctggactggagttgtcccggtgccctggagacccagtcactgccacctctcccctgcctggactcagcaggggaaagactggaggccctgctcctgccctttggctctgccagcacccccgaccagccctatatctcctcctccaccttcaagatcatccctgagaagacctcgagccccgagtgggtgcccttggggctgtcctgggagcctccagcaggcccctgggccactccactggcaggactaccgtcctggagtgagggtgaggcttcccgggtagggcgtgcttccaccagcctctcgagggtccggttgagggcctccacgccatcggccagacgctggctctgctcggccagccgctgcagcagcaggttttgctgggccatgagtgtgctctgctgctgggcccaggaggacagcagggcgccctgctgccggtgggagtccagcagctgctgctcaaatgcggacgtttcagatgctgccgctggggtcctcctggagggcaagggaggtgctggcgccgaagagggcggggaaggctggaaggcccccatgagtgtggttgctggtggggtggaggctggggaagcaggtggggagggtgaggaggtgggtgcgtggaagactcctcgtaagtccagggggtcaggttcaggcaggctgggcccttccagggacctcaggggcagccacaagcagctgggggtctcgtcctcctcatcagttggcaggggctccgtggtctggccctcgccttggggaccgtgggcagaaaaggtctctgccaccatgcgctccacaggtgtgaggaggaggccgggggcggggccgccctccgccagcttcttgcgcacagcacctcgcaggtcccgccacttgtgcttgaggtcccccaggtcgcggcggcagtagcccagcgcgttcactgcctgcaggatgcggctccacacgcggtgctttcgggcaggtgtgccccgcagcgccccgaacagcagcgggtagtggcgccgcaccctctgcaccagcacctccgtctcctgggggctgaagttgggcttgcgtgtcttggtgcgggagtgggggcccggccgcaggggtgtggagcccggcccggcacccagcagcagggctgccgcggccggctcggggctgcagctctgctggcagatggctttgctgctgctggacccaacagcttctccttgctctgacaccatggaggccaagtccttgatgatctgattcacatccagcaagttgctctccatctgcaggatggcctcctcccgcagccggatggcctccaggtcctcttcagtgatgtccgggagcagcgcctgctcctggccctgccacatgttgtcactcccgttaaagaccttctcatcatcagccagctcggcaaacggggcctggggactctgctgtttactgcccctctgcgccatgggaagcagcgctctggacttttctgcaattttcttctgcaccactccatagcactgaatggcatctgagagctgggttttcagccggtccagctgaggacgctcctgctgcagacgctcctgcgggcaggagctgcgcagcagctcggccatctgcttcacggagctggcgctggctgcaatggtcttgttggtctcctgctgtgccgtgtgcaggctgtcccgaagctcctgcgtgtcactcggtgtccctaaggactgaaggctccgctccaaggaggtcacactggagttgattcggaagacgttggccgacatctcctggaacagctcctggaggttgcacggatcgacctgggtggctctgggcggctccagactgaagccctcggagggcagggcctggcaagagaaggtcttggccaccacctgctccacgggcgtgagagccagggcctggggcttgccggaaccagggctggggccatgggccgccttccggaggtcgcccagcttgcgccgcacgacggctcgtaggtcccgccacttgtgcttcaggtccacaacgtcgcggcgacagtagcccagcgcattcacggcctgcaggatgcggctccacacgcggtacctgcgagtgggctcggccttcagcagccccgtgccaaacagcagctggtggtgcttgctcaccttggacaccagcacctcggtctcctgcgggcagaagttgggcttcctcttcttggcccgggtagtgctgggccccgccatccggccatggggcccagcagccgagtccttcctcgggccaatggtgggtgatgaggtgggctccggcatccggctgccttcaggggcaaccccaggccctcgcttcctggcccttgggacaataggcgtgcctgctggccccagatcaccttccccgtccttccccacacagcggttctgcagcttgctctctggcgacgggcaggggaaatggcggattccatactcggtccaacatctagcgcactctaggggctgacagccttgtctcgaaggtcccccgaaagggccacggctccccaggccacctccacgggcgatggatccgtatgacatcttcttacagatggcagggccagcagcctccacactgagctggggtctgaacagcgcgcgaggacccgccgaggggctcatgtgcccgcgggccggtccccgaaatgcggcgctctcgcggggctgcggctcagggtc

SEQ ID NO: 15664 - RNA, 4295 nt, Homo sapiens
  source 1..4295: mol_type = other RNA
gctgggattacaggcatgagccactgtgcccaggccatggtgggtatttttaatggacaagaacccagaatgaagatctacagaggcttcctggaggtggtgggactgaggtcatctggtttggcaggatggaaggccagctttcccagggtggaaccatcagagtggaggccccgcccagaaccaacagcagcaccatgcgcacccatagaaggggtagcctggagggaggccaggcgtgcgcagaaggcagctggacatgtggctacacctcaggttctttcatagacaagttactgacacattgctggctccaggggaaaacgcaaaacgaggaaaaggcccctctccctgctctcagggatgctgtagtcttttgactctcggctgtgccagagcttccccggaagctcctgggaccagcatgcctcccactcaagccagtcagccagcatcttgctcctgggacaggctttgggccatgggagccaggcagaggccccagactagccaaggcccgggctggtcccacctcccgctcctgctcgctcccgacggctgcctaggctggggggctgcagactgtgccctgccgcgcagggactggagatgtggcagccccgccaagggatctcccaagagtcaaaggaggtaatggaggaagaaggatctgaagacgcagggaagtgcccaggcccccgcagggaggctgaaagcagcggtgcctgccacgcccgagaagcaggctccaactcacgtgctcgtcagcagccgcactgctgcctgctttgtcattttatgcttatgtaaaaaaatactttttgcaagaaaaatctacaggtacaaaatgtcatcccagccccatacagtaccaagtaatatataggcatatatatatatatatatatatttatgtatttataacagaaaattggatagaaattattccaggcatatgggatgtggttcccctgggccagaaccacgtagggcagaggagccctgccctccaagtgtgcatgcccaccaaagggacaggggctttcaggagtcacaccagatcacgcttgggacctttttagagcctggctgagccaccctttccagagttccagtgagcagggggcccctcagtgcatcttccccacctcccctgcttccagggacgctgggctgcagacttcgcagctgctgccacatggggttggagcctccaacagcatcatccctgagtagacctggtccactgagtcccacaggtcggctctctgcagcctttccctgcaggtcaccaccctctacaggcaatggcaaggacgcgacatcacaggtagacagcccacatcctctcatccttccggtctcctggactggagttgtcccggtgccctggagacccagtcactgccacctctcccctgcctggactcagcaggggaaagactggaggccctgctcctgccctttggctctgccagcacccccgaccagccctatatctcctcctccaccttcaagatcatccctgagaagacctcgagccccgagtgggtgcccttggggctgtcctgggagcctccagcaggcccctgggccactccactggcaggactaccgtcctggagtgagggtgaggcttcccgggtagggcgtgcttccaccagcctctcgagggtccggttgagggcctccacgccatcggccagacgctggctctgctcggccagccgctgcagcagcaggttttgctgggccatgagtgtgctctgctgctgggcccaggaggacagcagggcgccctgctgccggtgggagtccagcagctgctgctcaaatgcggacgtttcagatgctgccgctggggtcctcctggagggcaagggaggtgctggcgccgaagagggcggggaaggctggaaggcccccatgagtgtggttgctggtggggtggaggctggggaagcaggtggggagggtgaggaggtgggtgcgtggaagactcctcgtaagtccagggggtcaggttcaggcaggctgggcccttccagggacctcaggggcagccacaagcagctgggggtctcgtcctcctcatcagttggcaggggctccgtggtctggccctcgccttggggaccgtgggcagaaaaggtctctgccaccatgcgctccacaggtgtgaggaggaggccgggggcggggccgccctccgccagcttcttgcgcacagcacctcgcaggtcccgccacttgtgcttgaggtcccccaggtcgcggcggcagtagcccagcgcgttcactgcctgcaggatgcggctccacacgcggtgctttcgggcaggtgtgccccgcagcgccccgaacagcagcgggtagtggcgccgcaccctctgcaccagcacctccgtctcctgggggctgaagttgggcttgcgtgtcttggtgcgggagtgggggcccggccgcaggggtgtggagcccggcccggcacccagcagcagggctgccgcggccggctcggggctgcagctctgctggcagatggctttgctgctgctggacccaacagcttctccttgctctgacaccatggaggccaagtccttgatgatctgattcacatccagcaagttgctctccatctgcaggatggcctcctcccgcagccggatggcctccaggtcctcttcagtgatgtccgggagcagcgcctgctcctggccctgccacatgttgtcactcccgttaaagaccttctcatcatcagccagctcggcaaacggggcctggggactctgctgtttactgcccctctgcgccatgggaagcagcgctctggacttttctgcaattttcttctgcaccactccatagcactgaatggcatctgagagctgggttttcagccggtccagctgaggacgctcctgctgcagacgctcctgcgggcaggagctgcgcagcagctcggccatctgcttcacggagctggcgctggctgcaatggtcttgttggtctcctgctgtgccgtgtgcctggtgaggtttttctgaagctgaatgtattcgggtggaaggaccacccttcctcctgagactgggtccctcctacactgcagggctggaaagccttttccctgacgaaatgatggcggccgtggatgaaggtatattctttaaatgtccttagttggcaacttcgtcaatgtggaggaaatatagaactggcaaccacgttggtctcaaaagttatttttaaatgttaacagtccatgatatgggagcatcagaggggccacagaaggctctagataagccatgccaagcaggctagacccacagctggccatgcagggagggtcagaaaagcactaaggcgagtttccagacctaagagctaaggccggcccaggggagagccaaggtgccgggatactcggtcctcagaccaggacagtctcctactccacgctggggtcccctctcctctccgaggcccacagcgggtggtgtcggtcttcagctaaccaggccgggcggcccaggatgcgcacatgagggccagggtccggacgtgcccatcccacctggccctcgtgacctaacccaggagtgggccagtggcactaagatctaagcacagcagcttcactgggaacctgcccaccacactgaagagacgggagagccacagacccggcccagagttacacaagttatctgcatcaacagggccctctgagaggccacacgtttcctgagcccgagcaccccagagcccaggtgtgaccagcaggtccacagtccctcactgaggtctgaccgtgcaaatacgcgtgggtgtgaggaaggctggagggaacaccgacatgctaacagcagctcccaggcatcctgcgtccaaattccctatcatgagcctacgtcactgtcacatcagaaaacacttaagtttcagttttataaaagagcttaaaaaaaaaggctaagaatagaactgccctgaacatctgcaaagggtgctccgcagctggtgcgtgaggctgtgtggcaggcgcctgcggattttgaacggagccgccgtgaggaggagcagagactccagcaccctccacccttgtgggagccgtggccctcccggcctcctcagttctggccctttcagggtgcaaggctggtgtggccaccagttctgcacaggggagtgcgaggacaacgtcccagtgcagtggcctggggctggctggggtccttggagctgcgggcatcccgctcactgcagggcgggacacagg

SEQ ID NO: 15665 - RNA, 4153 nt, Homo sapiens
  source 1..4153: mol_type = other RNA
gctgggattacaggcatgagccactgtgcccaggccatggtgggtatttttaatggacaagaacccagaatgaagatctacagaggcttcctggaggtggtgggactgaggtcatctggtttggcaggatggaaggccagctttcccagggtggaaccatcagagtggaggccccgcccagaaccaacagcagcaccatgcgcacccatagaaggggtagcctggagggaggccaggcgtgcgcagaaggcagctggacatgtggctacacctcaggttctttcatagacaagttactgacacattgctggctccaggggaaaacgcaaaacgaggaaaaggcccctctccctgctctcagggatgctgtagtcttttgactctcggctgtgccagagcttccccggaagctcctgggaccagcatgcctcccactcaagccagtcagccagcatcttgctcctgggacaggctttgggccatgggagccaggcagaggccccagactagccaaggcccgggctggtcccacctcccgctcctgctcgctcccgacggctgcctaggctggggggctgcagactgtgccctgccgcgcagggactggagatgtggcagccccgccaagggatctcccaagagtcaaaggaggtaatggaggaagaaggatctgaagacgcagggaagtgcccaggcccccgcagggaggctgaaagcagcggtgcctgccacgcccgagaagcaggctccaactcacgtgctcgtcagcagccgcactgctgcctgctttgtcattttatgcttatgtaaaaaaatactttttgcaagaaaaatctacaggtacaaaatgtcatcccagccccatacagtaccaagtaatatataggcatatatatatatatatatatatttatgtatttataacagaaaattggatagaaattattccaggcatatgggatgtggttcccctgggccagaaccacgtagggcagaggagccctgccctccaagtgtgcatgcccaccaaagggacaggggctttcaggagtcacaccagatcacgcttgggacctttttagagcctggctgagccaccctttccagagttccagtgagcagggggcccctcagtgcatcttccccacctcccctgcttccagggacgctgggctgcagacttcgcagctgctgccacatggggttggagcctccaacagcatcatccctgagtagacctggtccactgagtcccacaggtcggctctctgcagcctttccctgcaggtcaccaccctctacaggcaatggcaaggacgcgacatcacaggtagacagcccacatcctctcatccttccggtctcctggactggagttgtcccggtgccctggagacccagtcactgccacctctcccctgcctggactcagcaggggaaagactggaggccctgctcctgccctttggctctgccagcacccccgaccagccctatatctcctcctccaccttcaagatcatccctgagaagacctcgagccccgagtgggtgcccttggggctgtcctgggagcctccagcaggcccctgggccactccactggcaggactaccgtcctggagtgagggtgaggcttcccgggtagggcgtgcttccaccagcctctcgagggtccggttgagggcctccacgccatcggccagacgctggctctgctcggccagccgctgcagcagcaggttttgctgggccatgagtgtgctctgctgctgggcccaggaggacagcagggcgccctgctgccggtgggagtccagcagctgctgctcaaatgcggacgtttcagatgctgccgctggggtcctcctggagggcaagggaggtgctggcgccgaagagggcggggaaggctggaaggcccccatgagtgtggttgctggtggggtggaggctggggaagcaggtggggagggtgaggaggtgggtgcgtggaagactcctcgtaagtccagggggtcaggttcaggcaggctgggcccttccagggacctcaggggcagccacaagcagctgggggtctcgtcctcctcatcagttggcaggggctccgtggtctggccctcgccttggggaccgtgggcagaaaaggtctctgccaccatgcgctccacaggtgtgaggaggaggccgggggcggggccgccctccgccagcttcttgcgcacagcacctcgcaggtcccgccacttgtgcttgaggtcccccaggtcgcggcggcagtagcccagcgcgttcactgcctgcaggatgcggctccacacgcggtgctttcgggcaggtgtgccccgcagcgccccgaacagcagcgggtagtggcgccgcaccctctgcaccagcacctccgtctcctgggggctgaagttgggcttgcgtgtcttggtgcgggagtgggggcccggccgcaggggtgtggagcccggcccggcacccagcagcagggctgccgcggccggctcggggctgcagctctgctggcagatggctttgctgctgctggacccaacagcttctccttgctctgacaccatggaggccaagtccttgatgatctgattcacatccagcaagttgctctccatctgcaggatggcctcctcccgcagccggatggcctccaggtcctcttcagtgatgtccgggagcagcgcctgctcctggccctgccacatgttgtcactcccgttaaagaccttctcatcatcagccagctcggcaaacggggcctggggactctgtttactgcccctctgcgccatgggaagcagcgctctggacttttctgcaattttcttctgcaccactccatagcactgaatggcatctgagagctgggttttcagccggtccagctgaggacgctcctgctgcagacgctcctgcgggcaggagctgcgcagcagctcggccatctgcttcacggagctggcgctggctgcaatggtcttgttggtctcctgctgtgccgtgtgcaggctgtcccgaagctcctgcgtgtcactcggtgtccctaaggactgaaggctccgctccaaggaggtcacactggagttgattcggaagacgttggccgacatctcctggaacagctcctggaggttgcacggatcgacctgggtggctctgggcggctccagactgaagccctcggagggcagggcctggcaagagaaggtcttggccaccacctgctccacgggcgtgagagccagggcctggggcttgccggaaccagggctggggccatgggccgccttccggaggtcgcccagcttgcgccgcacgacggctcgtaggtcccgccacttgtgcttcaggtccacaacgtcgcggcgacagtagcccagcgcattcacggcctgcaggatgcggctccacacgcggtacctgcgagtgggctcggccttcagcagccccgtgccaaacagcagctggtggtgcttgctcaccttggacaccagcacctcggtctcctgcgggcagaagttgggcttcctcttcttggcccgggtagtgctgggccccgccatccggccatggggcccagcagccgagtccttcctcgggccaatggtgggtgatgaggtgggctccggcatccggctgccttcaggggcaaccccaggccctcgcttcctggcccttgggacaataggcgtgcctgctggccccagatcaccttccccgtccttccccacacagcggttctgcagcttgctctctggcgacgggcaggggaaatggcggattccatactcggtccaacatctagcgcactctaggggctgacagccttgtctcgaaggtcccccgaaagggccacggctccccaggccacctccacgggcgatggatccgtatgacatcttcttacagatggcagggccagcagcctccacactgagctgggcctcggtggctcgcggaccgctccgggcgctcacggcgggcgaggcgggcggggcgggcacccaaacatcacgtgacggcccctcccgccgccggcgtgcgcgccccctcccgcaccagccaatggccgccggtcccggacgcgcgcggggactacccgccccagaggccccggcgcggagcc

SEQ ID NO: 15666 - RNA, 3005 nt, Homo sapiens
  source 1..3005: mol_type = other RNA
gctgggattacaggcatgagccactgtgcccaggccatggtgggtatttttaatggacaagaacccagaatgaagatctacagaggcttcctggaggtggtgggactgaggtcatctggtttggcaggatggaaggccagctttcccagggtggaaccatcagagtggaggccccgcccagaaccaacagcagcaccatgcgcacccatagaaggggtagcctggagggaggccaggcgtgcgcagaaggcagctggacatgtggctacacctcaggttctttcatagacaagttactgacacattgctggctccaggggaaaacgcaaaacgaggaaaaggcccctctccctgctctcagggatgctgtagtcttttgactctcggctgtgccagagcttccccggaagctcctgggaccagcatgcctcccactcaagccagtcagccagcatcttgctcctgggacaggctttgggccatgggagccaggcagaggccccagactagccaaggcccgggctggtcccacctcccgctcctgctcgctcccgacggctgcctaggctggggggctgcagactgtgccctgccgcgcagggactggagatgtggcagccccgccaagggatctcccaagagtcaaaggaggtaatggaggaagaaggatctgaagacgcagggaagtgcccaggcccccgcagggaggctgaaagcagcggtgcctgccacgcccgagaagcaggctccaactcacgtgctcgtcagcagccgcactgctgcctgctttgtcattttatgcttatgtaaaaaaatactttttgcaagaaaaatctacaggtacaaaatgtcatcccagccccatacagtaccaagtaatatataggcatatatatatatatatatatatttatgtatttataacagaaaattggatagaaattattccaggcatatgggatgtggttcccctgggccagaaccacgtagggcagaggagccctgccctccaagtgtgcatgcccaccaaagggacaggggctttcaggagtcacaccagatcacgcttgggacctttttagagcctggctgagccaccctttccagagttccagtgagcagggggcccctcagtgcatcttccccacctcccctgcttccagggacgctgggctgcagacttcgcagctgctgccacatggggttggagcctccaacagcatcatccctgagtagacctggtccactgagtcccacaggtcggctctctgcagcctttccctgcaggtcaccaccctctacaggcaatggcaaggacgcgacatcacaggtagacagcccacatcctctcatccttccggtctcctggactggagttgtcccggtgccctggagacccagtcactgccacctctcccctgcctggactcagcaggggaaagactggaggccctgctcctgccctttggctctgccagcacccccgaccagccctatatctcctcctccaccttcaagatcatccctgagaagacctcgagccccgagtgggtgcccttggggctgtcctgggagcctccagcaggcccctgggccactccactggcaggactaccgtcctggagtgagggtgaggcttcccgggtagggcgtgcttccaccagcctctcgagggtccggttgagggcctccacgccatcggccagacgctggctctgctcggccagccgctgcagcagcaggttttgctgggccatgagtgtgctctgctgctgggcccaggaggacagcagggcgccctgctgccggtgggagtccagcagctgctgctcaaatgcggacgtttcagatgctgccgctggggtcctcctggagggcaagggaggtgctggcgccgaagagggcggggaaggctggaaggcccccatgagtgtggttgctggtggggtggaggctggggaagcaggtggggagggtgaggaggtgggtgcgtggaagactcctcgtaagtccagggggtcaggttcaggcaggctgggcccttccagggacctcaggggcagccacaagcagctgggggtctcgtcctcctcatcagttggtgccggctggctccagccaggagctggcgggctgcctccgcatgcgaggacgcagcctcaaggctggcttcaatactatcaacagcttctccttgctctgacaccatggaggccaagtccttgatgatctgattcacatccagcaagttgctctccatctgcaggatggcctcctcccgcagccggatggcctccaggtcctcttcagtgatgtccgggagcagcgcctgctcctggccctgccacatgttgtcactcccgttaaagaccttctcatcatcagccagctcggcaaacggggcctggggactctgctgtttactgcccctctgcgccatgggaagcagcgctctggacttttctgcaattttcttctgcaccactccatagcactgaatggcatctgagagctgggttttcagccggtccagctgaggacgctcctgctgcagacgctccgggcaggagctgcgcagcagctcggccatctgcttcacggagctggcgctggctgcaatggtcttgttggtctcctgctgtgccgtgtgcaggctgtcccgaagctcctgcgtgtcactcggtgtccctaaggactgaaggctccgctccaaggaggtcacactggagttgattcggaagacgttggccgacatctcctggaacagctcctggaggttgcacggatcgacctgggtggctaggggctgacagccttgtctcgaaggtcccccgaaagggccacggctccccaggccacctccacgggcgatggatccgtatgacatcttcttacagatggcagggccagcagcctccacactgagctgggcctcggtggctcgcggaccgctccgggcgctcacggcgggcgaggcgggcggggcgggcacccaaacatcacgt

SEQ ID NO: 15667 - RNA, 3662 nt, Homo sapiens
  source 1..3662: mol_type = other RNA
gctgggattacaggcatgagccactgtgcccaggccatggtgggtatttttaatggacaagaacccagaatgaagatctacagaggcttcctggaggtggtgggactgaggtcatctggtttggcaggatggaaggccagctttcccagggtggaaccatcagagtggaggccccgcccagaaccaacagcagcaccatgcgcacccatagaaggggtagcctggagggaggccaggcgtgcgcagaaggcagctggacatgtggctacacctcaggttctttcatagacaagttactgacacattgctggctccaggggaaaacgcaaaacgaggaaaaggcccctctccctgctctcagggatgctgtagtcttttgactctcggctgtgccagagcttccccggaagctcctgggaccagcatgcctcccactcaagccagtcagccagcatcttgctcctgggacaggctttgggccatgggagccaggcagaggccccagactagccaaggcccgggctggtcccacctcccgctcctgctcgctcccgacggctgcctaggctggggggctgcagactgtgccctgccgcgcagggactggagatgtggcagccccgccaagggatctcccaagagtcaaaggaggtaatggaggaagaaggatctgaagacgcagggaagtgcccaggcccccgcagggaggctgaaagcagcggtgcctgccacgcccgagaagcaggctccaactcacgtgctcgtcagcagccgcactgctgcctgctttgtcattttatgcttatgtaaaaaaatactttttgcaagaaaaatctacaggtacaaaatgtcatcccagccccatacagtaccaagtaatatataggcatatatatatatatatatatatttatgtatttataacagaaaattggatagaaattattccaggcatatgggatgtggttcccctgggccagaaccacgtagggcagaggagccctgccctccaagtgtgcatgcccaccaaagggacaggggctttcaggagtcacaccagatcacgcttgggacctttttagagcctggctgagccaccctttccagagttccagtgagcagggggcccctcagtgcatcttccccacctcccctgcttccagggacgctgggctgcagacttcgcagctgctgccacatggggttggagcctccaacagcatcatccctgagtagacctggtccactgagtcccacaggtcggctctctgcagcctttccctgcaggtcaccaccctctacaggcaatggcaaggacgcgacatcacaggtagacagcccacatcctctcatccttccggtctcctggactggagttgtcccggtgccctggagacccagtcactgccacctctcccctgcctggactcagcaggggaaagactggaggccctgctcctgccctttggctctgccagcacccccgaccagccctatatctcctcctccaccttcaagatcatccctgagaagacctcgagccccgagtgggtgcccttggggctgtcctgggagcctccagcaggcccctgggccactccactggcaggactaccgtcctggagtgagggtgaggcttcccgggtagggcgtgcttccaccagcctctcgagggtccggttgagggcctccacgccatcggccagacgctggctctgctcggccagccgctgcagcagcaggttttgctgggccatgagtgtgctctgctgctgggcccaggaggacagcagggcgccctgctgccggtgggagtccagcagctgctgctcaaatgcggacgtttcagatgctgccgctggggtcctcctggagggcaagggaggtgctggcgccgaagagggcggggaaggctggaaggcccccatgagtgtggttgctggtggggtggaggctggggaagcaggtggggagggtgaggaggtgggtgcgtggaagactcctcgtaagtccagggggtcaggttcaggcaggctgggcccttccagggacctcaggggcagccacaagcagctgggggtctcgtcctcctcatcagttggtgccggctggctccagccaggagctggcgggctgcctccgcatgcgaggacgcagcctcaaggctggcttcaatactatcaacagcttctccttgctctgacaccatggaggccaagtccttgatgatctgattcacatccagcaagttgctctccatctgcaggatggcctcctcccgcagccggatggcctccaggtcctcttcagtgatgtccgggagcagcgcctgctcctggccctgccacatgttgtcactcccgttaaagaccttctcatcatcagccagctcggcaaacggggcctggggactctgtttactgcccctctgcgccatgggaagcagcgctctggacttttctgcaattttcttctgcaccactccatagcactgaatggcatctgagagctgggttttcagccggtccagctgaggacgctcctgctgcagacgctcctgcgggcaggagctgcgcagcagctcggccatctgcttcacggagctggcgctggctgcaatggtcttgttggtctcctgctgtgccgtgtgcaggctgtcccgaagctcctgcgtgtcactcggtgtccctaaggactgaaggctccgctccaaggaggtcacactggagttgattcggaagacgttggccgacatctcctggaacagctcctggaggttgcacggatcgacctgggtggctctgggcggctccagactgaagccctcggagggcagggcctggcaagagaaggtcttggccaccacctgctccacgggcgtgagagccagggcctggggcttgccggaaccagggctggggccatgggccgccttccggaggtcgcccagcttgcgccgcacgacggctcgtaggtcccgccacttgtgcttcaggtccacaacgtcgcggcgacagtagcccagcgcattcacggcctgcaggatgcggctccacacgcggtacctgcgagtgggctcggccttcagcagccccgtgccaaacagcagctggtggtgcttgctcaccttggacaccagcacctcggtctcctgcgggcagaagttgggcttcctcttcttggcccgggtagtgctgggccccgccatccggccatggggcccagcagccgagtccttcctcgggccaatggtgggtgatgaggtgggctccggcatccggctgccttcaggggcaaccccaggccctcgcttcctggcccttgggacaataggcgtgcctgctggccccagatcaccttccccgtccttccccacacagcggttctgcagcttgctctctggcgacgggcaggggaaatggcggattccatactcggtccaacatctagcgcactctaggggctgacagccttgtctcgaaggtcccccgaaagggccacggctccccaggccacctccacgggcgatggatccgtatgacatcttcttacagatggcagggccagcagcctccacactgagctgggcctcggtggctcgcggaccgctccgggcgctcacggcgggcgaggcgggcggggcgggcacccaaacatcacgt

SEQ ID NO: 15668 - RNA, 4579 nt, Homo sapiens
  source 1..4579: mol_type = other RNA
gctgggattacaggcatgagccactgtgcccagtcactgttctttatatacaaaaaagaatgtgtgaaatttttaaaatgtacattgcaaaagacgattattctactcaaaatttatttggtaagattttattaagactctaagttcaaacacccttcttgggaaaagctctacaggataaccacacatgctcaactacggggccagctgctgcagctgtgggaccccatcctgtggaagaggagagaggcactaaaaagatgaggtagccaggcctgtgcccacactacgagacctgcatcaccatggtgtgaggagcagcaacgtgggtcaactcggggctgggacgagatggaagagtaaaaggcctttcttcataggcctgcctattttatgaccaccagggtagacttttgtaattaaattaaggtccacatgactttagaaagacaaactaaaaaaccccaaccaaacgagtcctagctgtagctaactctgatttctgtaaattggatctgactttttctgcttacattcacttaaaatctcaaagactcaatgggtgtgaagtgctaacaccttgcggcaaaatctcaaattcatctgtgccaggccctctgcacagcagggctcagcagggcaggccagggctctggtccctggtcccttgctgggggaggtgttccatccggccagcgcccggccatgcagccacgtgactcaagcacgggaagtgcaggggcccagacacatccaggctaaagggcagtgactaggggagggctgaccccaagctgaacagggttctaaccaaacgctcaggagctcccaggtgacagcaaccacgccaccatgaacacaccactgggtctgtactggaatttgggggcctcaaggcttccaggtggcagcataaacagggaggtggggcaggataggaatgcccccctctgaggctcggcagccgggtggaatgaaccactccctctcattcagtgacagcacaggcaccctcctcattctgggctacccagatcttccagccctgtccctccaccccacctctcttagcctaagcagcactgagggcctggagtggtctctgtccaccccacccccacatgcggggagccttcccatacccctcagccccacagcaccagctccacccaccctctccagcctgagctcctgcacacaccccagctgccctcaccctgagctcagtgccctccttgctgaagggaacggctagtacaggaggagctggggcccaggggtctgactccatcaccaaggcaaagcccagagtggttgggctggcgtgagtgcaggctgggccctggtctgaaatgagtgtctttattgcttgtaccgtacaaatatgaagacgaggagaaaggccagtagggacggagaactgtcagataacaacatcgcacacagaggaaaaagaccctcacccacccgaaccaaccccacccctccccaccctgccatgaactgtgtagtacaggagatgggatagggagagcaaacccacaaaagctaaactccaaacacccagaggtgttgctacagggaggggaggcgtgggcagggcagctcatggatcacagtggggctcctcccactaggtcagcacccctcccccacaggatgaaatgctcgggccagggatggggcccaagcccacacaccatgcacactggaggacacgctgccctcacacaaacacacatgcacacacacccacgtgtgcctgcgtcccgccgacacacgcagtccgaggcacgcacaggagtcccacagcactgacatggacgtgcactcatgttcaaccttaaggctgcagaacgtggggccctggggagagggaggggtgaggggggcctaggagcctcccttttcagaggccccccaccccaataggtaccagagatgcccacccccacccctccctgaccaagtccatggggcccaatactgtccggtgtaagattgtaacagccaaggctggtggccctccacccccgcagaggagagggtgagcccagcccatagcccccagtggggccaggccaggcccagggtccagcgggaggtaaggccagctggaaggaagccctagtaaggcacggggctgggaggcaggcaggtttggccccaaatgttcctcctgcctcatccatagggtgaggacagtttggtggggaggaggccggaccaggaggcggcacccagcccggccactcctggttccccatggtacagatcctaggatctgactccattcaccagggagcagccctaacccccagccctgcagctcccaagggcccctgcctgcccctggacattattgcttttctgcccccatagggggacagcgggtgggggattggaccgccccgtgcctggccactccgagcctaggccacggggcctggaaggcagcaccactgtctgccgggtgtcgcgtcccaccagaaggcagccttcgtccagatgcagcagcgcggaggcagacaccagcacgacacccaggccagaaactcaggcaggccccaggcgccatgcttcacccctcactggggcttgtgtggattaaaacctgaatctccaaccgcccaacagcccaggcctgggcgggaggtggagtcttccaaatgcgagtctgggcacaaaggtgaggctggaggctggaggcaggggctgcaggggccgctggggtgcgtctgggaggggcctgaagaagaactggaaagggggtgaggaggtgggggtggggacacaaaccaaaaaggctaagtaaaaagttagggggaaaaaaccacccagcggtgatggcagcgagcgtgcgtcctctgcgtgggcagactgctcactcgcggatgctggccgagtaggagaactgggggaagtgggtccgctggtccagctccagtaagcccaggctgtcatagcggtcagggggtgtgattgtgatggactgggcggtaaattcatcatcgaagtaccttgtgtcgacctcggacgtgacctgaggtttgaagggtggcaggagcttcttctggaccacgtcctgccagttgatgctgaggaagaacctgtgctccatgacctccttggcatcgctgggccccccaccaagcctctgcttggggtccttcttaagcagcccagcaagcagggacttggcctcggggctgagcgtgcgcgggaagcggatctcttccatgaggatgagctcgaagaggcgctcgtggtcctggttgtagaagggcaggcggccgcacatcatctcgtacatgaccacacccagcccccaccagtccacggcccggccatagtcattgtcctccagcacctcaggcgccaggtactccggggtcccacagaaggttttcatggtggccccgtcactgatgccctctttgcagaggccaaagtcagtgatcttgatgtggccatctttgtccagcatgaggttttccagcttgatgtcgcggtataccacgtcccgcgagtgcaagtactcaagagccgagacaatctctgcaccataaaaccgggcccgctcctctgtgaagacacgctcccgggacaggtggaagaacagctcacccccgttggcatactccatcacaaagcacaggcggtcgtgggtctggaaggcatacttcagcgcagtgaggaacgggtgcctggtgttctggaggacccggctctcggtgactgtgtgagcgacttcatccttggcaatgatgacttccttccgcaggatcttcatggcgtagtagcggccagtggccttctcccgcaccaggatgactttgccaaaggttcccttgccaaggagtttgagatagtcgaagtcattcatggtcactttagcccgtgccttgctgaccgccacttccatctcctcagtcgtggaggagtcactgggggagccacacttgtagtccatggggtcctcgcctggggcccgctgcttgaggctgttggcgaccatctggatggcccgcatccactcctccctctcgtctggagaatccacgtggaaggtcctctcgatgactgtggtccactgcaggcagcgtatgacaaaggtgttgggtcgcggcctctcggtcttcatcagctggcattctgctacggagaagttgtttaaggggggtagagtctgatcaggggcctcgggcctctccttgtacccaatgaaggagccgtcgctcttcagcaggaagtaccgtggcctccaggtcttgatgtattcaccacgcttgtggagccagccttctttgatgacagacacctcattcatggtggcagcgtggtacgctgtcacctagctcgggacagctcagggcagcaggacatgcaggaggcaccgtggacagggcacagtctgtcaccggcagccgcccagcctctccggcggggctctacccccgcccatcgccacgctgcgctggttccctttccttgtgtttcccggcagcggcaacggcgccggcagcggcagcggcggcggcgacgcctcctccgaggcaggcccaacggctagcacggc

SEQ ID NO: 15669 - RNA, 4542 nt, Homo sapiens
  source 1..4542: mol_type = other RNA
gctgggattacaggcatgagccactgtgcccagtcactgttctttatatacaaaaaagaatgtgtgaaatttttaaaatgtacattgcaaaagacgattattctactcaaaatttatttggtaagattttattaagactctaagttcaaacacccttcttgggaaaagctctacaggataaccacacatgctcaactacggggccagctgctgcagctgtgggaccccatcctgtggaagaggagagaggcactaaaaagatgaggtagccaggcctgtgcccacactacgagacctgcatcaccatggtgtgaggagcagcaacgtgggtcaactcggggctgggacgagatggaagagtaaaaggcctttcttcataggcctgcctattttatgaccaccagggtagacttttgtaattaaattaaggtccacatgactttagaaagacaaactaaaaaaccccaaccaaacgagtcctagctgtagctaactctgatttctgtaaattggatctgactttttctgcttacattcacttaaaatctcaaagactcaatgggtgtgaagtgctaacaccttgcggcaaaatctcaaattcatctgtgccaggccctctgcacagcagggctcagcagggcaggccagggctctggtccctggtcccttgctgggggaggtgttccatccggccagcgcccggccatgcagccacgtgactcaagcacgggaagtgcaggggcccagacacatccaggctaaagggcagtgactaggggagggctgaccccaagctgaacagggttctaaccaaacgctcaggagctcccaggtgacagcaaccacgccaccatgaacacaccactgggtctgtactggaatttgggggcctcaaggcttccaggtggcagcataaacagggaggtggggcaggataggaatgcccccctctgaggctcggcagccgggtggaatgaaccactccctctcattcagtgacagcacaggcaccctcctcattctgggctacccagatcttccagccctgtccctccaccccacctctcttagcctaagcagcactgagggcctggagtggtctctgtccaccccacccccacatgcggggagccttcccatacccctcagccccacagcaccagctccacccaccctctccagcctgagctcctgcacacaccccagctgccctcaccctgagctcagtgccctccttgctgaagggaacggctagtacaggaggagctggggcccaggggtctgactccatcaccaaggcaaagcccagagtggttgggctggcgtgagtgcaggctgggccctggtctgaaatgagtgtctttattgcttgtaccgtacaaatatgaagacgaggagaaaggccagtagggacggagaactgtcagataacaacatcgcacacagaggaaaaagaccctcacccacccgaaccaaccccacccctccccaccctgccatgaactgtgtagtacaggagatgggatagggagagcaaacccacaaaagctaaactccaaacacccagaggtgttgctacagggaggggaggcgtgggcagggcagctcatggatcacagtggggctcctcccactaggtcagcacccctcccccacaggatgaaatgctcgggccagggatggggcccaagcccacacaccatgcacactggaggacacgctgccctcacacaaacacacatgcacacacacccacgtgtgcctgcgtcccgccgacacacgcagtccgaggcacgcacaggagtcccacagcactgacatggacgtgcactcatgttcaaccttaaggctgcagaacgtggggccctggggagagggaggggtgaggggggcctaggagcctcccttttcagaggccccccaccccaataggtaccagagatgcccacccccacccctccctgaccaagtccatggggcccaatactgtccggtgtaagattgtaacagccaaggctggtggccctccacccccgcagaggagagggtgagcccagcccatagcccccagtggggccaggccaggcccagggtccagcgggaggtaaggccagctggaaggaagccctagtaaggcacggggctgggaggcaggcaggtttggccccaaatgttcctcctgcctcatccatagggtgaggacagtttggtggggaggaggccggaccaggaggcggcacccagcccggccactcctggttccccatggtacagatcctaggatctgactccattcaccagggagcagccctaacccccagccctgcagctcccaagggcccctgcctgcccctggacattattgcttttctgcccccatagggggacagcgggtgggggattggaccgccccgtgcctggccactccgagcctaggccacggggcctggaaggcagcaccactgtctgccgggtgtcgcgtcccaccagaaggcagccttcgtccagatgcagcagcgcggaggcagacaccagcacgacacccaggccagaaactcaggcaggccccaggcgccatgcttcacccctcactggggcttgtgtggattaaaacctgaatctccaaccgcccaacagcccaggcctgggcgggaggtggagtcttccaaatgcgagtctgggcacaaaggtgaggctggaggctggaggcaggggctgcaggggccgctggggtgcgtctgggaggggcctgaagaagaactggaaagggggtgaggaggtgggggtggggacacaaaccaaaaaggctaagtaaaaagttagggggaaaaaaccacccagcggtgatggcagcgagcgtgcgtcctctgcgtgggcagactgctcactcgcggatgctggccgagtaggagaactgggggaagtgggtccgctggtccagctccagtaagcccaggctgtcatagcggtcagggggtgtgattgtgatggactgggcggtaaattcatcatcgaagtaccttgtgtcgacctcggacgtgacctgaggtttgaagggtggcaggagcttcttctggaccacgtcctgccagttgatgctgaggaagaacctgtgctccatgacctccttggcatcgctgggccccccaccaagcctctgcttggggtccttcttaagcagcccagcaagcagggacttggcctcggggctgagcgtgcgcgggaagcggatctcttccatgaggatgagctcgaagaggcgctcgtggtcctggttgtagaagggcaggcggccgcacatcatctcgtacatgaccacacccagcccccaccagtccacggcccggccatagtcattgtcctccagcacctcaggcgccaggtactccggggtcccacagaaggttttcatggtggccccgtcactgatgccctctttgcagaggccaaagtcagtgatcttgatgtggccatctttgtccagcatgaggttttccagcttgatgtcgcggtataccacgtcccgcgagtgcaagtactcaagagccgagacaatctctgcaccataaaaccgggcccgctcctctgtgaagacacgctcccgggacaggtggaagaacagctcacccccgttggcatactccatcacaaagcacaggcggtcgtgggtctggaaggcatacttcagcgcagtgaggaacgggtgcctggtgttctggaggacccggctctcggtgactgtgtgagcgacttcatccttggcaatgatgacttccttccgcaggatcttcatggcgtagtagcggccagtggccttctcccgcaccaggatgactttgccaaaggttcccttgccaaggagtttgagatagtcgaagtcattcatggtcactttagcccgtgccttgctgaccgccacttccatctcctcagtcgtggaggagtcactgggggagccacacttgtagtccatggggtcctcgcctggggcccgctgcttgaggctgttggcgaccatctggatggcccgcatccactcctccctctcgtctggagaatccacgtggaaggtcctctcgatgactgtggtccactgcaggcagcgtatgacaaaggtgttgggtcgcggcctctcggtcttcatcagctggcattctgctacggagaagttgtttaaggggggtagagtctgatcaggggcctcgggcctctccttgtacccaatgaaggagccgtcgctcttcagcaggaagtaccgtggcctccaggtcttgatgtattcacctcattcatggtggcagcgtggtacgctgtcacctagctcgggacagctcagggcagcaggacatgcaggaggcaccgtggacagggcacagtctgtcaccggcagccgcccagcctctccggcggggctctacccccgcccatcgccacgctgcgctggttccctttccttgtgtttcccggcagcggcaacggcgccggcagcggcagcggcggcggcgacgcctcctccgaggcaggcccaacggctagcacggc

SEQ ID NO: 15670 - RNA, 4449 nt, Homo sapiens
  source 1..4449: mol_type = other RNA
gctgggattacaggcatgagccactgtgcccagtcactgttctttatatacaaaaaagaatgtgtgaaatttttaaaatgtacattgcaaaagacgattattctactcaaaatttatttggtaagattttattaagactctaagttcaaacacccttcttgggaaaagctctacaggataaccacacatgctcaactacggggccagctgctgcagctgtgggaccccatcctgtggaagaggagagaggcactaaaaagatgaggtagccaggcctgtgcccacactacgagacctgcatcaccatggtgtgaggagcagcaacgtgggtcaactcggggctgggacgagatggaagagtaaaaggcctttcttcataggcctgcctattttatgaccaccagggtagacttttgtaattaaattaaggtccacatgactttagaaagacaaactaaaaaaccccaaccaaacgagtcctagctgtagctaactctgatttctgtaaattggatctgactttttctgcttacattcacttaaaatctcaaagactcaatgggtgtgaagtgctaacaccttgcggcaaaatctcaaattcatctgtgccaggccctctgcacagcagggctcagcagggcaggccagggctctggtccctggtcccttgctgggggaggtgttccatccggccagcgcccggccatgcagccacgtgactcaagcacgggaagtgcaggggcccagacacatccaggctaaagggcagtgactaggggagggctgaccccaagctgaacagggttctaaccaaacgctcaggagctcccaggtgacagcaaccacgccaccatgaacacaccactgggtctgtactggaatttgggggcctcaaggcttccaggtggcagcataaacagggaggtggggcaggataggaatgcccccctctgaggctcggcagccgggtggaatgaaccactccctctcattcagtgacagcacaggcaccctcctcattctgggctacccagatcttccagccctgtccctccaccccacctctcttagcctaagcagcactgagggcctggagtggtctctgtccaccccacccccacatgcggggagccttcccatacccctcagccccacagcaccagctccacccaccctctccagcctgagctcctgcacacaccccagctgccctcaccctgagctcagtgccctccttgctgaagggaacggctagtacaggaggagctggggcccaggggtctgactccatcaccaaggcaaagcccagagtggttgggctggcgtgagtgcaggctgggccctggtctgaaatgagtgtctttattgcttgtaccgtacaaatatgaagacgaggagaaaggccagtagggacggagaactgtcagataacaacatcgcacacagaggaaaaagaccctcacccacccgaaccaaccccacccctccccaccctgccatgaactgtgtagtacaggagatgggatagggagagcaaacccacaaaagctaaactccaaacacccagaggtgttgctacagggaggggaggcgtgggcagggcagctcatggatcacagtggggctcctcccactaggtcagcacccctcccccacaggatgaaatgctcgggccagggatggggcccaagcccacacaccatgcacactggaggacacgctgccctcacacaaacacacatgcacacacacccacgtgtgcctgcgtcccgccgacacacgcagtccgaggcacgcacaggagtcccacagcactgacatggacgtgcactcatgttcaaccttaaggctgcagaacgtggggccctggggagagggaggggtgaggggggcctaggagcctcccttttcagaggccccccaccccaataggtaccagagatgcccacccccacccctccctgaccaagtccatggggcccaatactgtccggtgtaagattgtaacagccaaggctggtggccctccacccccgcagaggagagggtgagcccagcccatagcccccagtggggccaggccaggcccagggtccagcgggaggtaaggccagctggaaggaagccctagtaaggcacggggctgggaggcaggcaggtttggccccaaatgttcctcctgcctcatccatagggtgaggacagtttggtggggaggaggccggaccaggaggcggcacccagcccggccactcctggttccccatggtacagatcctaggatctgactccattcaccagggagcagccctaacccccagccctgcagctcccaagggcccctgcctgcccctggacattattgcttttctgcccccatagggggacagcgggtgggggattggaccgccccgtgcctggccactccgagcctaggccacggggcctggaaggcagcaccactgtctgccgggtgtcgcgtcccaccagaaggcagccttcgtccagatgcagcagcgcggaggcagacaccagcacgacacccaggccagaaactcaggcaggccccaggcgccatgcttcacccctcactggggcttgtgtggattaaaacctgaatctccaaccgcccaacagcccaggcctgggcgggaggtggagtcttccaaatgcgagtctgggcacaaaggtgaggctggaggctggaggcaggggctgcaggggccgctggggtgcgtctgggaggggcctgaagaagaactggaaagggggtgaggaggtgggggtggggacacaaaccaaaaaggctaagtaaaaagttagggggaaaaaaccacccagcggtgatggcagcgagcgtgcgtcctctgcgtgggcagactgctcactcgcggatgctggccgagtaggagaactgggggaagtgggtccgctggtccagctccagtaagcccaggctgtcatagcggtcagggggtgtgattgtgatggactgggcggtaaattcatcatcgaagtaccttgtgtcgacctcggacgtgacctgaggtttgaagggtggcaggagcttcttctggaccacgtcctgccagttgatgctgaggaagaacctgtgctccatgacctccttggcatcgctgggccccccaccaagcctctgcttggggtccttcttaagcagcccagcaagcagggacttggcctcggggctgagcgtgcgcgggaagcggatctcttccatgaggatgagctcgaagaggcgctcgtggtcctggttgtagaagggcaggcggccgcacatcatctcgtacatgaccacacccagcccccaccagtccacggcccggccatagtcattgtcctccagcacctcaggcgccaggtactccggggtcccacagaaggttttcatggtggccccgtcactgatgccctctttgcagaggccaaagtcagtgatcttgatgtggccatctttgtccagcatgaggttttccagcttgatgtcgcggtataccacgtcccgcgagtgcaagtactcaagagccgagacaatctctgcaccataaaaccgggcccgctcctctgtgaagacacgctcccgggacaggtggaagaacagctcacccccgttggcatactccatcacaaagcacaggcggtcgtgggtctggaaggcatacttcagcgcagtgaggaacgggtgcctggtgttctggaggacccggctctcggtgactgtgtgagcgacttcatccttggcaatgatgacttccttccgcaggatcttcatggcgtagtagcggccagtggccttctcccgcaccaggatgactttgccaaaggttcccttgccaaggagtttgagatagtcgaagtcattcatggtcactttagcccgtgccttgctgaccgccacttccatctcctcagtcgtggaggagtcactgggggagccacacttgtagtccatggggtcctcgcctggggcccgctgcttgaggctgttggcgaccatctggatggcccgcatccactcctccctctcgtctggagaatccacgtggaaggtcctctcgatgactgtggtccactgcaggcagcgtatgacaaaggtgttgggtcgcggcctctcggtcttcatcagctggcattctgctacggagaagttgtttaaggggggtagagtctgatcaggggcctcgggcctctccttgtacccaatgaaggagccgtcgctcttcagcaggaagtaccgtggcctccaggtcttgatgtattcacctgtcaccggcagccgcccagcctctccggcggggctctacccccgcccatcgccacgctgcgctggttccctttccttgtgtttcccggcagcggcaacggcgccggcagcggcagcggcggcggcgacgcctcctccgaggcaggcccaacggctagcacggc

SEQ ID NO: 15671 - RNA, 4285 nt, Homo sapiens
  source 1..4285: mol_type = other RNA
gctgggattacaggcatgagccactgtgcccagtcactgttctttatatacaaaaaagaatgtgtgaaatttttaaaatgtacattgcaaaagacgattattctactcaaaatttatttggtaagattttattaagactctaagttcaaacacccttcttgggaaaagctctacaggataaccacacatgctcaactacggggccagctgctgcagctgtgggaccccatcctgtggaagaggagagaggcactaaaaagatgaggtagccaggcctgtgcccacactacgagacctgcatcaccatggtgtgaggagcagcaacgtgggtcaactcggggctgggacgagatggaagagtaaaaggcctttcttcataggcctgcctattttatgaccaccagggtagacttttgtaattaaattaaggtccacatgactttagaaagacaaactaaaaaaccccaaccaaacgagtcctagctgtagctaactctgatttctgtaaattggatctgactttttctgcttacattcacttaaaatctcaaagactcaatgggtgtgaagtgctaacaccttgcggcaaaatctcaaattcatctgtgccaggccctctgcacagcagggctcagcagggcaggccagggctctggtccctggtcccttgctgggggaggtgttccatccggccagcgcccggccatgcagccacgtgactcaagcacgggaagtgcaggggcccagacacatccaggctaaagggcagtgactaggggagggctgaccccaagctgaacagggttctaaccaaacgctcaggagctcccaggtgacagcaaccacgccaccatgaacacaccactgggtctgtactggaatttgggggcctcaaggcttccaggtggcagcataaacagggaggtggggcaggataggaatgcccccctctgaggctcggcagccgggtggaatgaaccactccctctcattcagtgacagcacaggcaccctcctcattctgggctacccagatcttccagccctgtccctccaccccacctctcttagcctaagcagcactgagggcctggagtggtctctgtccaccccacccccacatgcggggagccttcccatacccctcagccccacagcaccagctccacccaccctctccagcctgagctcctgcacacaccccagctgccctcaccctgagctcagtgccctccttgctgaagggaacggctagtacaggaggagctggggcccaggggtctgactccatcaccaaggcaaagcccagagtggttgggctggcgtgagtgcaggctgggccctggtctgaaatgagtgtctttattgcttgtaccgtacaaatatgaagacgaggagaaaggccagtagggacggagaactgtcagataacaacatcgcacacagaggaaaaagaccctcacccacccgaaccaaccccacccctccccaccctgccatgaactgtgtagtacaggagatgggatagggagagcaaacccacaaaagctaaactccaaacacccagaggtgttgctacagggaggggaggcgtgggcagggcagctcatggatcacagtggggctcctcccactaggtcagcacccctcccccacaggatgaaatgctcgggccagggatggggcccaagcccacacaccatgcacactggaggacacgctgccctcacacaaacacacatgcacacacacccacgtgtgcctgcgtcccgccgacacacgcagtccgaggcacgcacaggagtcccacagcactgacatggacgtgcactcatgttcaaccttaaggctgcagaacgtggggccctggggagagggaggggtgaggggggcctaggagcctcccttttcagaggccccccaccccaataggtaccagagatgcccacccccacccctccctgaccaagtccatggggcccaatactgtccggtgtaagattgtaacagccaaggctggtggccctccacccccgcagaggagagggtgagcccagcccatagcccccagtggggccaggccaggcccagggtccagcgggaggtaaggccagctggaaggaagccctagtaaggcacggggctgggaggcaggcaggtttggccccaaatgttcctcctgcctcatccatagggtgaggacagtttggtggggaggaggccggaccaggaggcggcacccagcccggccactcctggttccccatggtacagatcctaggatctgactccattcaccagggagcagccctaacccccagccctgcagctcccaagggcccctgcctgcccctggacattattgcttttctgcccccatagggggacagcgggtgggggattggaccgccccgtgcctggccactccgagcctaggccacggggcctggaaggcagcaccactgtctgccgggtgtcgcgtcccaccagaaggcagccttcgtccagatgcagcagcgcggaggcagacaccagcacgacacccaggccagaaactcaggcaggccccaggcgccatgcttcacccctcactggggcttgtgtggattaaaacctgaatctccaaccgcccaacagcccaggcctgggcgggaggtggagtcttccaaatgcgagtctgggcacaaaggtgaggctggaggctggaggcaggggctgcaggggccgctggggtgcgtctgggaggggcctgaagaagaactggaaagggggtgaggaggtgggggtggggacacaaaccaaaaaggctaagtaaaaagttagggggaaaaaaccacccagcggtgatggcagcgagcgtgcgtcctctgcgtgggcagactgctcactcgcggatgctggccgagtaggagaactgggggaagtgggtccgctggtccagctccagtaagcccaggctgtcatagcggtcagggggtgtgattgtgatggactgggcggtaaattcatcatcgaagtaccttgtgtcgacctcggacgtgacctgaggtttgaagggtggcaggagcttcttctggaccacgtcctgccagttgatgctgaggaagaacctgtgctccatgacctccttggcatcgctgggccccccaccaagcctctgcttggggtccttcttaagcagcccagcaagcagggacttggcctcggggctgagcgtgcgcgggaagcggatctcttccatgaggatgagctcgaagaggcgctcgtggtcctggttgtagaagggcaggcggccgcacatcatctcgtacatgaccacacccagcccccaccagtccacggcccggccatagtcattgtcctccagcaccttgatgtcgcggtataccacgtcccgcgagtgcaagtactcaagagccgagacaatctctgcaccataaaaccgggcccgctcctctgtgaagacacgctcccgggacaggtggaagaacagctcacccccgttggcatactccatcacaaagcacaggcggtcgtgggtctggaaggcatacttcagcgcagtgaggaacgggtgcctggtgttctggaggacccggctctcggtgactgtgtgagcgacttcatccttggcaatgatgacttccttccgcaggatcttcatggcgtagtagcggccagtggccttctcccgcaccaggatgactttgccaaaggttcccttgccaaggagtttgagatagtcgaagtcattcatggtcactttagcccgtgccttgctgaccgccacttccatctcctcagtcgtggaggagtcactgggggagccacacttgtagtccatggggtcctcgcctggggcccgctgcttgaggctgttggcgaccatctggatggcccgcatccactcctccctctcgtctggagaatccacgtggaaggtcctctcgatgactgtggtccactgcaggcagcgtatgacaaaggtgttgggtcgcggcctctcggtcttcatcagctggcattctgctacggagaagttgtttaaggggggtagagtctgatcaggggcctcgggcctctccttgtacccaatgaaggagccgtcgctcttcagcaggaagtaccgtggcctccaggtcttgatgtattcaccacgcttgtggagccagccttctttgatgacagacacctcattcatggtggcagcgtggtacgctgtcacctagctcgggacagctcagggcagcaggacatgcaggaggcaccgtggacagggcacagt

SEQ ID NO: 15672 - RNA, 3235 nt, Homo sapiens
  source 1..3235: mol_type = other RNA
gctgggattacaggcatgagccactgtgcccatctctgggtaggtttgcgttgtgaggcctgatgccctgttcttctcttctcctttccgaagtccgtggccctctggtggcctctgtggcttcttgagctaatctcacccactgtgggcctcaggttccgctcccctaaacatggctgcagagggcaacaccatctcccagcacccttctaagagtgtggctgctaaactcttcagggacatagtactagagtgtgacaaagaccccataggaagtgtcacacaggtgcgaggcttcacacagtgccgctcatttccttccagaaatacctccatactcttttactatcctgagggtggggcaccccacatttctctggcatttgatctcccttcccccacagcagctcttctcaccaagatgcctttccttggcacggcgcttgcagcccaagcagggctgaaggagaggggcctgagtctcaggggtgttcctccccttggagagctctgggctggcagcatcttgctaaggggttgtcagcctcccaacctgggacaaggacagctcctcctcctctgtgtatggtaactacaggggtggaaggcaaggcagagaagttgacgggaggtagcaagagtgggagccggtggcataatttagatctgaggcctttaagaaaaatgctcagaaacaatcatcctacccagtgctaaatatcagatgagtcagcctctgggcagctgtcaccttcctcccccaaattccctggcaaagcagggaggctggcttggggctgcctctctgactctgacagcagttggaacccacagctaccctgcggtccccctcttgcccccaatcccaggatgctcgcttccattttactctacttttagggaaggagccagggatgggcctcagtgttccctccctactcccgaagggacagtatttgtccccagtcctttctcctgccgatgcttttggatttaggaagtgatgccttgaggacatgggcatctcccacccttcgtgctcaccctcgcaatagtggatgtgcctggagggtacatttctgaagaactaccagagctgagaagaaaaagcagactgcatagcttagcgcagattcacgcaaagccacttgtgcattccagagccagggccatgtggttcggcccacatgttggcagtaagcatgttgttccagccaggtgagtcagcagacatgggatgttcgtttatttgggcaaatgtgtctcgttagggtcattctgaaaagaagcccagtgtgcagtcattagcccctggggtagcgttgctactaagtggttggggagaagtcagggaagaggaagaggtggcgttccccagcctcacccgtggagaccccagcgaagcgggggcaggcaggcactgctggaggagcgaaggccaggtggacacgaggacagattccagaggcttggttttattgtgcagttttctttgtcctcaatgagatgccataagctgtggtggcactatacacagtcacagaacaggaagaaccaccgggtgggggctgggggttgggaaaagccatttcctgagaagtgtccggctcctgggtctcactccatggcttgcctcaggccccgcagaagtccctgagaaggcaggcctgcggggcagggggctgtctgaggggctcaggcaccagccagcaggggctggcactgatgggcgaggggaggaagtgcctcccttagaaacttgggccaaaccctgtgcagctctgggactccaccccacctgacttggaggctgtgggtcagagctctggaagctcttgggagcttgggacagcctgagagggtcttgtcctcctttgtagccctctccactgtgggtggaggcagggaggggcagcagggccatgcttttagcttccttaggcagggagggatgatgaaccctcatcctttacctccttctccaaccctccactagcgctgctttcctggtcaaacctgcatcttcactgggtcatgccccaaggcctctgagggacttccacagtggtaaggagggctgccctttttatttttttttggttgtggctgagaatgctggagatgctcagttctctccctcacaaggtaggccacaaattcttggtggtgccctcacatctggggtcttcaggcaccagccatgcctgccgaggagtgctgtcaggacagaccatgtccgtgctaggcccaggcacagcccaaccactcctcatccaagtctctcccaggtttctggtcccgatgggcaaggatgacccctccagtggctggtaccccaccatcccactacccctcacatgctctcactctccatcaggtccccaatcctggcttccctcttcacgaactctcaaagaaaaggaaggataaaacctaaataaaccagacagaagcagctctggaacaaaaagtacaaaaagacagccagaggtgtgcggagagggtgaggtggccgcgtggacgtgggtagataatcgcatgcagcactggaactcctgatgaggggtggggtccccacttctcctcaaggtttgagggattggggggagggggtcagctgactcagagaagtaggatctctgcactggaacttgaggcttcctgtctcctccatgggccccaccagtcacagggacatgaaatccgtggcctggaggagggagagggagagcaggagcagcagcagccacgaggtgttctgagccagcaggctgatgccctcacacttgaccagtttgtctctgagcactgtgacgttctgggaggagatgggtggggaatggccagagtggtggagtgcacacgtgtaggtgccctcgtccttgctagtgaaggcggataagtagaggaccttcatgttgtatttgctggtgaagttggttcgggagcggtatgtgtgctcaggcacccccacagtgccaaagagcacgtgcttctttgtctcacgggtcaggctgaactcgtactggatgggtgaactgctggtattctcatggcggcagtccagacgaaggctctggtccactaggcaggccgttaggctggtcaccttctgccctcgggagacctgcaagacgcgaggtcacccggcagattccctctagctcgccatcctccatcctctccccgcagtttcatccgtcctcctccccgcctctgcgagctgggtttgggg

SEQ ID NO: 15673 - RNA, 4148 nt, Homo sapiens
  source 1..4148: mol_type = other RNA
gctgggattacaggcatgagccactgtgcccatctctgggtaggtttgcgttgtgaggcctgatgccctgttcttctcttctcctttccgaagtccgtggccctctggtggcctctgtggcttcttgagctaatctcacccactgtgggcctcaggttccgctcccctaaacatggctgcagagggcaacaccatctcccagcacccttctaagagtgtggctgctaaactcttcagggacatagtactagagtgtgacaaagaccccataggaagtgtcacacaggtgcgaggcttcacacagtgccgctcatttccttccagaaatacctccatactcttttactatcctgagggtggggcaccccacatttctctggcatttgatctcccttcccccacagcagctcttctcaccaagatgcctttccttggcacggcgcttgcagcccaagcagggctgaaggagaggggcctgagtctcaggggtgttcctccccttggagagctctgggctggcagcatcttgctaaggggttgtcagcctcccaacctgggacaaggacagctcctcctcctctgtgtatggtaactacaggggtggaaggcaaggcagagaagttgacgggaggtagcaagagtgggagccggtggcataatttagatctgaggcctttaagaaaaatgctcagaaacaatcatcctacccagtgctaaatatcagatgagtcagcctctgggcagctgtcaccttcctcccccaaattccctggcaaagcagggaggctggcttggggctgcctctctgactctgacagcagttggaacccacagctaccctgcggtccccctcttgcccccaatcccaggatgctcgcttccattttactctacttttagggaaggagccagggatgggcctcagtgttccctccctactcccgaagggacagtatttgtccccagtcctttctcctgccgatgcttttggatttaggaagtgatgccttgaggacatgggcatctcccacccttcgtgctcaccctcgcaatagtggatgtgcctggagggtacatttctgaagaactaccagagctgagaagaaaaagcagactgcatagcttagcgcagattcacgcaaagccacttgtgcattccagagccagggccatgtggttcggcccacatgttggcagtaagcatgttgttccagccaggtgagtcagcagacatgggatgttcgtttatttgggcaaatgtgtctcgttagggtcattctgaaaagaagcccagtgtgcagtcattagcccctggggtagcgttgctactaagtggttggggagaagtcagggaagaggaagaggtggcgttccccagcctcacccgtggagaccccagcgaagcgggggcaggcaggcactgctggaggagcgaaggccaggtggacacgaggacagattccagaggcttggttttattgtgcagttttctttgtcctcaatgagatgccataagctgtggtggcactatacacagtcacagaacaggaagaaccaccgggtgggggctgggggttgggaaaagccatttcctgagaagtgtccggctcctgggtctcactccatggcttgcctcaggccccgcagaagtccctgagaaggcaggcctgcggggcagggggctgtctgaggggctcaggcaccagccagcaggggctggcactgatgggcgaggggaggaagtgcctcccttagaaacttgggccaaaccctgtgcagctctgggactccaccccacctgacttggaggctgtgggtcagagctctggaagctcttgggagcttgggacagcctgagagggtcttgtcctcctttgtagccctctccactgtgggtggaggcagggaggggcagcagggccatgcttttagcttccttaggcagggagggatgatgaaccctcatcctttacctccttctccaaccctccactagcgctgctttcctggtcaaacctgcatcttcactgggtcatgccccaaggcctctgagggacttccacagtggtaaggagggctgccctttttatttttttttggttgtggctgagaatgctggagatgctcagttctctccctcacaaggtaggccacaaattcttggtggtgccctcacatctggggtcttcaggcaccagccatgcctgccgaggagtgctgtcaggacagaccatgtccgtgctaggcccaggcacagcccaaccactcctcatccaagtctctcccaggtttctggtcccgatgggcaaggatgacccctccagtggctggtaccccaccatcccactacccctcacatgctctcactctccatcaggtccccaatcctggcttccctcttcacgaactctcaaagaaaaggaaggataaaacctaaataaaccagacagaagcagctctggaacaaaaagtacaaaaagacagccagaggtgtgcggagagggtgaggtggccgcgtggacgtgggtagataatcgcatgcagcactggaactcctgatgaggggtggggtccccacttctcctcaaggtttgagggattggggggagggggtcagctgactcagagaagtaggatctctgcactggaacttgaggcttcctgtctcctccatgggccccaccagtcacagggacatgaaatccgtggcctggaggagggagagggagagcaggagcagcagcagccacgaggtgttctgagccagcaggctgatgccctcacacttgaccagtttgtctctgagcactgtgacgttctgggaggagatgggtggggaatggccagagtggtggagtgcacacgtgtaggtgccctcgtccttgctagtgaaggcggataagtagaggaccttcatgttgtatttgctggtgaagttggttcgggagcggtatgtgtgctcaggcacccccacagtgccaaagagcacgtgcttctttgtctcacgggtcaggctgaactcgtactggatgggtgaactgctggtattctcatggcggcagtccagacgaaggctctggtccactaggcaggccgttaggctggtcaccttctgccctcgggagacctgcaagactgttagcaggagagcgatgctgatggccaggttcatggttctgggatctcagtcctggatcgggttatgatgggggttaagaaaaacaaccaacatctggcgatgactgcttcatatacgtgagacacaaatccctaagtcactcgccatccccagtggatggctagataccattcaccatagctaaggatgctcccagatagggagcatctattcctatctggataggacacaagctaatcgtgttcctggaggagagaaagacatagtgatctccgattgtatgtgagccaaggatgcttcccaatgtccagctctctggagttcctgggactgcagttttccagcccagtttcaatagccaccctggataggctgtctgcctggtctttttttgttttttgcagccttggctgaaccaacccttggcgaggcgacgcggagccggtagtctagcctatctgcagagcagtgctcgcccaggagaggccacagaaggggcgtgcacccgcgagagcgcgcagggcattgcctcggttgagtgcgcccgggtgcgcagggcgcaccactagacgagttcagggtccctggcgctcagccccttgacgggtgaggctaggatcccgcggcggctgcagctacaatcaatgctctctctgtcccggggtggagctgctgccctgagccagatccaggaggaaggggggtcggcatctggcttttgaatcgaggactcttgtttgagatgttgtgcgggcttgggatctaggaggggaagggggagcaatggccagagcaagaaagggaagaaatgggtctggggctggagagggtagaagagccaggggaggggtggagagcggctggggaggtgcagtctgtattcatttcctctggtctgtgtcctcaggcggctccagacccagagaaggtctgctcttcctccctctcaagcccccggcgggcctcatccttaatccatttccgtattccaatcctctcctttcccaaa

SEQ ID NO: 15674 - RNA, 3284 nt, Homo sapiens
  source 1..3284: mol_type = other RNA
gctgggattacaggcatgagccactgtgcccatctctgggtaggtttgcgttgtgaggcctgatgccctgttcttctcttctcctttccgaagtccgtggccctctggtggcctctgtggcttcttgagctaatctcacccactgtgggcctcaggttccgctcccctaaacatggctgcagagggcaacaccatctcccagcacccttctaagagtgtggctgctaaactcttcagggacatagtactagagtgtgacaaagaccccataggaagtgtcacacaggtgcgaggcttcacacagtgccgctcatttccttccagaaatacctccatactcttttactatcctgagggtggggcaccccacatttctctggcatttgatctcccttcccccacagcagctcttctcaccaagatgcctttccttggcacggcgcttgcagcccaagcagggctgaaggagaggggcctgagtctcaggggtgttcctccccttggagagctctgggctggcagcatcttgctaaggggttgtcagcctcccaacctgggacaaggacagctcctcctcctctgtgtatggtaactacaggggtggaaggcaaggcagagaagttgacgggaggtagcaagagtgggagccggtggcataatttagatctgaggcctttaagaaaaatgctcagaaacaatcatcctacccagtgctaaatatcagatgagtcagcctctgggcagctgtcaccttcctcccccaaattccctggcaaagcagggaggctggcttggggctgcctctctgactctgacagcagttggaacccacagctaccctgcggtccccctcttgcccccaatcccaggatgctcgcttccattttactctacttttagggaaggagccagggatgggcctcagtgttccctccctactcccgaagggacagtatttgtccccagtcctttctcctgccgatgcttttggatttaggaagtgatgccttgaggacatgggcatctcccacccttcgtgctcaccctcgcaatagtggatgtgcctggagggtacatttctgaagaactaccagagctgagaagaaaaagcagactgcatagcttagcgcagattcacgcaaagccacttgtgcattccagagccagggccatgtggttcggcccacatgttggcagtaagcatgttgttccagccaggtgagtcagcagacatgggatgttcgtttatttgggcaaatgtgtctcgttagggtcattctgaaaagaagcccagtgtgcagtcattagcccctggggtagcgttgctactaagtggttggggagaagtcagggaagaggaagaggtggcgttccccagcctcacccgtggagaccccagcgaagcgggggcaggcaggcactgctggaggagcgaaggccaggtggacacgaggacagattccagaggcttggttttattgtgcagttttctttgtcctcaatgagatgccataagctgtggtggcactatacacagtcacagaacaggaagaaccaccgggtgggggctgggggttgggaaaagccatttcctgagaagtgtccggctcctgggtctcactccatggcttgcctcaggccccgcagaagtccctgagaaggcaggcctgcggggcagggggctgtctgaggggctcaggcaccagccagcaggggctggcactgatgggcgaggggaggaagtgcctcccttagaaacttgggccaaaccctgtgcagctctgggactccaccccacctgacttggaggctgtgggtcagagctctggaagctcttgggagcttgggacagcctgagagggtcttgtcctcctttgtagccctctccactgtgggtggaggcagggaggggcagcagggccatgcttttagcttccttaggcagggagggatgatgaaccctcatcctttacctccttctccaaccctccactagcgctgctttcctggtcaaacctgcatcttcactgggtcatgccccaaggcctctgagggacttccacagtggtaaggagggctgccctttttatttttttttggttgtggctgagaatgctggagatgctcagttctctccctcacaaggtaggccacaaattcttggtggtgccctcacatctggggtcttcaggcaccagccatgcctgccgaggagtgctgtcaggacagaccatgtccgtgctaggcccaggcacagcccaaccactcctcatccaagtctctcccaggtttctggtcccgatgggcaaggatgacccctccagtggctggtaccccaccatcccactacccctcacatgctctcactctccatcaggtccccaatcctggcttccctcttcacgaactctcaaagaaaaggaaggataaaacctaaataaaccagacagaagcagctctggaacaaaaagtacaaaaagacagccagaggtgtgcggagagggtgaggtggccgcgtggacgtgggtagataatcgcatgcagcactggaactcctgatgaggggtggggtccccacttctcctcaaggtttgagggattggggggagggggtcagctgactcagagaagtaggatctctgcactggaacttgaggcttcctgtctcctccatgggccccaccagtcacagggacatgaaatccgtggcctggaggagggagagggagagcaggagcagcagcagccacgaggtgttctgagccagcaggctgatgccctcacacttgaccagtttgtctctgagcactgtgacgttctgggaggagatgggtggggaatggccagagtggtggagtgcacacgtgtaggtgccctcgtccttgctagtgaaggcggataagtagaggaccttcatgttgtatttgctggtgaagttggttcgggagcggtatgtgtgctcaggcacccccacagtgccaaagagcacgtgcttctttgtctcacgggtcaggctgaactcgtactggatgggtgaactgctggtattctcatggcggcagtccagacgaaggctctggtccactaggcaggccgttaggctggtcaccttctgccctcgggagacctgcaagactgttagcaggagagcgatgctgatggccaggttcatggttctgggatctcagtcctggatctgatgcattccagacacactggctctggcttctgtctgcctcttcatggcagcgcactccttcctgcttaacagctttctgattctg

SEQ ID NO: 15675 - RNA, 3256 nt, Homo sapiens
  source 1..3256: mol_type = other RNA
gctgggattacaggcatgagccactgtgcccatctctgggtaggtttgcgttgtgaggcctgatgccctgttcttctcttctcctttccgaagtccgtggccctctggtggcctctgtggcttcttgagctaatctcacccactgtgggcctcaggttccgctcccctaaacatggctgcagagggcaacaccatctcccagcacccttctaagagtgtggctgctaaactcttcagggacatagtactagagtgtgacaaagaccccataggaagtgtcacacaggtgcgaggcttcacacagtgccgctcatttccttccagaaatacctccatactcttttactatcctgagggtggggcaccccacatttctctggcatttgatctcccttcccccacagcagctcttctcaccaagatgcctttccttggcacggcgcttgcagcccaagcagggctgaaggagaggggcctgagtctcaggggtgttcctccccttggagagctctgggctggcagcatcttgctaaggggttgtcagcctcccaacctgggacaaggacagctcctcctcctctgtgtatggtaactacaggggtggaaggcaaggcagagaagttgacgggaggtagcaagagtgggagccggtggcataatttagatctgaggcctttaagaaaaatgctcagaaacaatcatcctacccagtgctaaatatcagatgagtcagcctctgggcagctgtcaccttcctcccccaaattccctggcaaagcagggaggctggcttggggctgcctctctgactctgacagcagttggaacccacagctaccctgcggtccccctcttgcccccaatcccaggatgctcgcttccattttactctacttttagggaaggagccagggatgggcctcagtgttccctccctactcccgaagggacagtatttgtccccagtcctttctcctgccgatgcttttggatttaggaagtgatgccttgaggacatgggcatctcccacccttcgtgctcaccctcgcaatagtggatgtgcctggagggtacatttctgaagaactaccagagctgagaagaaaaagcagactgcatagcttagcgcagattcacgcaaagccacttgtgcattccagagccagggccatgtggttcggcccacatgttggcagtaagcatgttgttccagccaggtgagtcagcagacatgggatgttcgtttatttgggcaaatgtgtctcgttagggtcattctgaaaagaagcccagtgtgcagtcattagcccctggggtagcgttgctactaagtggttggggagaagtcagggaagaggaagaggtggcgttccccagcctcacccgtggagaccccagcgaagcgggggcaggcaggcactgctggaggagcgaaggccaggtggacacgaggacagattccagaggcttggttttattgtgcagttttctttgtcctcaatgagatgccataagctgtggtggcactatacacagtcacagaacaggaagaaccaccgggtgggggctgggggttgggaaaagccatttcctgagaagtgtccggctcctgggtctcactccatggcttgcctcaggccccgcagaagtccctgagaaggcaggcctgcggggcagggggctgtctgaggggctcaggcaccagccagcaggggctggcactgatgggcgaggggaggaagtgcctcccttagaaacttgggccaaaccctgtgcagctctgggactccaccccacctgacttggaggctgtgggtcagagctctggaagctcttgggagcttgggacagcctgagagggtcttgtcctcctttgtagccctctccactgtgggtggaggcagggaggggcagcagggccatgcttttagcttccttaggcagggagggatgatgaaccctcatcctttacctccttctccaaccctccactagcgctgctttcctggtcaaacctgcatcttcactgggtcatgccccaaggcctctgagggacttccacagtggtaaggagggctgccctttttatttttttttggttgtggctgagaatgctggagatgctcagttctctccctcacaaggtaggccacaaattcttggtggtgccctcacatctggggtcttcaggcaccagccatgcctgccgaggagtgctgtcaggacagaccatgtccgtgctaggcccaggcacagcccaaccactcctcatccaagtctctcccaggtttctggtcccgatgggcaaggatgacccctccagtggctggtaccccaccatcccactacccctcacatgctctcactctccatcaggtccccaatcctggcttccctcttcacgaactctcaaagaaaaggaaggataaaacctaaataaaccagacagaagcagctctggaacaaaaagtacaaaaagacagccagaggtgtgcggagagggtgaggtggccgcgtggacgtgggtagataatcgcatgcagcactggaactcctgatgaggggtggggtccccacttctcctcaaggtttgagggattggggggagggggtcagctgactcagagaagtaggatctctgcactggaacttgaggcttcctgtctcctccatgggccccaccagtcacagggacatgaaatccgtggcctggaggagggagagggagagcaggagcagcagcagccacgaggtgttctgagccagcaggctgatgccctcacacttgaccagtttgtctctgagcactgtgacgttctgggaggagatgggtggggaatggccagagtggtggagtgcacacgtgtaggtgccctcgtccttgctagtgaaggcggataagtagaggaccttcatgttgtatttgctggtgaagttggttcgggagcggtatgtgtgctcaggcacccccacagtgccaaagagcacgtgcttctttgtctcacgggtcaggctgaactcgtactggatgggtgaactgctggtattctcatggcggcagtccagacgaaggctctggtccactaggcaggccgttaggctggtcaccttctgccctcgggagacctgcaagactgttagcaggagagcgatgctgatggccaggttcatggttctgggatctcagtcctggatctggactggggtcttccgctgctgcagcctcctccagacgcgccgccgcctccggttgct

SEQ ID NO: 15676 - RNA, 3205 nt, Homo sapiens
  source 1..3205: mol_type = other RNA
gctgggattacaggcatgagccactgtgcccatctctgggtaggtttgcgttgtgaggcctgatgccctgttcttctcttctcctttccgaagtccgtggccctctggtggcctctgtggcttcttgagctaatctcacccactgtgggcctcaggttccgctcccctaaacatggctgcagagggcaacaccatctcccagcacccttctaagagtgtggctgctaaactcttcagggacatagtactagagtgtgacaaagaccccataggaagtgtcacacaggtgcgaggcttcacacagtgccgctcatttccttccagaaatacctccatactcttttactatcctgagggtggggcaccccacatttctctggcatttgatctcccttcccccacagcagctcttctcaccaagatgcctttccttggcacggcgcttgcagcccaagcagggctgaaggagaggggcctgagtctcaggggtgttcctccccttggagagctctgggctggcagcatcttgctaaggggttgtcagcctcccaacctgggacaaggacagctcctcctcctctgtgtatggtaactacaggggtggaaggcaaggcagagaagttgacgggaggtagcaagagtgggagccggtggcataatttagatctgaggcctttaagaaaaatgctcagaaacaatcatcctacccagtgctaaatatcagatgagtcagcctctgggcagctgtcaccttcctcccccaaattccctggcaaagcagggaggctggcttggggctgcctctctgactctgacagcagttggaacccacagctaccctgcggtccccctcttgcccccaatcccaggatgctcgcttccattttactctacttttagggaaggagccagggatgggcctcagtgttccctccctactcccgaagggacagtatttgtccccagtcctttctcctgccgatgcttttggatttaggaagtgatgccttgaggacatgggcatctcccacccttcgtgctcaccctcgcaatagtggatgtgcctggagggtacatttctgaagaactaccagagctgagaagaaaaagcagactgcatagcttagcgcagattcacgcaaagccacttgtgcattccagagccagggccatgtggttcggcccacatgttggcagtaagcatgttgttccagccaggtgagtcagcagacatgggatgttcgtttatttgggcaaatgtgtctcgttagggtcattctgaaaagaagcccagtgtgcagtcattagcccctggggtagcgttgctactaagtggttggggagaagtcagggaagaggaagaggtggcgttccccagcctcacccgtggagaccccagcgaagcgggggcaggcaggcactgctggaggagcgaaggccaggtggacacgaggacagattccagaggcttggttttattgtgcagttttctttgtcctcaatgagatgccataagctgtggtggcactatacacagtcacagaacaggaagaaccaccgggtgggggctgggggttgggaaaagccatttcctgagaagtgtccggctcctgggtctcactccatggcttgcctcaggccccgcagaagtccctgagaaggcaggcctgcggggcagggggctgtctgaggggctcaggcaccagccagcaggggctggcactgatgggcgaggggaggaagtgcctcccttagaaacttgggccaaaccctgtgcagctctgggactccaccccacctgacttggaggctgtgggtcagagctctggaagctcttgggagcttgggacagcctgagagggtcttgtcctcctttgtagccctctccactgtgggtggaggcagggaggggcagcagggccatgcttttagcttccttaggcagggagggatgatgaaccctcatcctttacctccttctccaaccctccactagcgctgctttcctggtcaaacctgcatcttcactgggtcatgccccaaggcctctgagggacttccacagtggtaaggagggctgccctttttatttttttttggttgtggctgagaatgctggagatgctcagttctctccctcacaaggtaggccacaaattcttggtggtgccctcacatctggggtcttcaggcaccagccatgcctgccgaggagtgctgtcaggacagaccatgtccgtgctaggcccaggcacagcccaaccactcctcatccaagtctctcccaggtttctggtcccgatgggcaaggatgacccctccagtggctggtaccccaccatcccactacccctcacatgctctcactctccatcaggtccccaatcctggcttccctcttcacgaactctcaaagaaaaggaaggataaaacctaaataaaccagacagaagcagctctggaacaaaaagtacaaaaagacagccagaggtgtgcggagagggtgaggtggccgcgtggacgtgggtagataatcgcatgcagcactggaactcctgatgaggggtggggtccccacttctcctcaaggtttgagggattggggggagggggtcagctgactcagagaagtaggatctctgcactggaacttgaggcttcctgtctcctccatgggccccaccagtcacagggacatgaaatccgtggcctggaggagggagagggagagcaggagcagcagcagccacgaggtgttctgagccagcaggctgatgccctcacacttgaccagtttgtctctgagcactgtgacgttctgggaggagatgggtggggaatggccagagtggtggagtgcacacgtgtaggtgccctcgtccttgctagtgaaggcggataagtagaggaccttcatgttgtatttgctggtgaagttggttcgggagcggtatgtgtgctcaggcacccccacagtgccaaagagcacgtgcttctttgtctcacgggtcaggctgaactcgtactggatgggtgaactgctggtattctcatggcggcagtccagacgaaggctctggtccactgttagcaggagagcgatgctgatggccaggttcatggttctgggatctcagtcctggatctggactggggtcttccgctgctgcagcctcctccagacgcgccgccgcctccggttgct

SEQ ID NO: 15677 - RNA, 2926 nt, Homo sapiens
  source 1..2926: mol_type = other RNA
gctgggattacaggcatgagccactgtgcccatgcccggcccaacttacgtttcatctaatgaccttattaagtgttcacttttcaaaggatcttttaacttcttctgaatgaacattagtcagctgcccctcccactagccaatctttagccctgagcacacatgggtataaaaacaatggaaaacaatcaaatttaatagtatcctaagtctcaacccaagaggaacaattagtagtaacactgattgagctgcttcaccacctttccccacaacccacctccatgtcaccatctgctattccactgacttggaggccaacgatataacctgccccacaacactctaaaacagctacctacttttatctcaaaagtactgacagaaggctccattagcagcaaacagacctatgaacacaaggtcctctacgctaggaaagcattactctttgaaatggggctatatttacaaattttatttttttatcccaaaaatacatataaatgaaaacctgctcttcaaatgcagggaggcctttgcctaacattgtcatatgaaaatcagtatcagctctttaacacacaatttacatatatacatacatacacactatatgtaagcagcaaatactttgctacttacacatattcctctggtggaaaactaggacactgggaaattcccctgctttccaaccttgggaaggtaaatacaacctctctcaacaactttttaaaggatgaaatgtgtagaaacatgtaaacaacacaacctgctttagatctatacatgttattagaataaagaaagaacgctgtcacatcagtgacagtttatttctcaaagaaaaaaagagataacatttgaataaaaatgcaaaactgaagtacagttaatatgatcaaaattgttgtgtacatgctccatggagaaatcaggaattctttcacaaagaacagatccacagccaatttcagtcacttgtgatgctgaatcagcacccactggtagcaaccaggatccttctgtacagtcacgggcttgagcaggtgccataaagcatctgtttaagttaaacagtcaataatgtttactgactgcagtacattcccaccccccaaaaaaataagtgcaaaatcaacttctaagctcaagagctcaaacaagtcaaagctttggtatatactggaggttgttttggtgataaccaaagcctagtaagattctctgctcaggggttcgccccaaaagaaaaacacctggtccacaaagcttaacacctatataaataaagtaactgtacaaagagaacaagccatgatttccccttaaccaagggtttatagtttcctaggcagcagttctgaaagcaccaactaaaaccacaacacttctactaaaacacggtgtgttgtaattggtgagactgttctgaaaacaaatgcctgcaggcatgtggccaaggtgccacagaaaaagtttaacaaacattagtcagtgtattcaaatggtaacacaatctggtcagcaacagaggaaagacttaaggcagtaagaggcattacagagagcaccatagtgctggacccaccaccatagtgctctctgagtcaatcaaagacttccaagaaggaaaccgtgtatcaatagtttgggttcttagtttgctagctgtcagacacttcttcctcctcctcctcatcctcgtcatctttcctgtctatttcagaagtgtccgacgactcatggagcaagacgtattctctgctactgaatccaaatttgagtacatccttttcttttagttcatagtatctctgtggctcaatacgtttgttgtttaagaaggttccattgcctgagccaaggtcaatgatgtagggcttcactcttcggccaactgtgccatcagcacgggtatattccacaagccgatattgaaagaccgcatgctgctttgaacaagacgggtgatcaattggaatgtctgcaatgcggcggtgtcgacccagtaggtacgcactctgtcgatgtatgtacatgactggaagcacctcatcatttttaaatgggtagagacgccaccgttttttggggatacgtgcttctgggggctcactatatttaatgactacaccccggaaagtgttggtgtcctcaagaagtgccccagaaagttcaaagcttggtttttctttagcgggcacctctttttctttgttgttgccaccaggccgaggaaccaactcctgagactcactgccgccaccaccaacgtcattcctctggcgatgctcccgtcgcctggcattataaaactcccgctcttcttcctgagcctgcaggttctgagtgtctcgatcccgtccctgaccctgcccactcccaggcctctcgttagacgttctcctttggtgggaatggccccggtgtctgtcccggtcactgttcctagctctcctgtgttcctgttctgatggttccctgtgctgccgatcctcccgtcctctccggggatgatcctcacgctcctgcttcactttgactgttgagtggtgaggacttcggtttctcttactgcgaggagacttgcttcttctccctgaggccttgtttttctttttgggtggggaccggctaactcctcgggctcggttcccgcggtggcccgagcgggccggctcgctggtcggcggagacgggctaccaccggagtggtccggacggcggtgggcgggaggtgcgacttctgggctgagacgctcctgcttcaccaccacccccgccggcagcaccacgtccccgtcccggtgtcttcgccggctccctcgctcccgttcgctcttcaccgccttcattctgtgattttggctgggcgaaagaaaacagatcagttgagctcctctagctggaggaaatgac

SEQ ID NO: 15678 - RNA, 2178 nt, Homo sapiens
  source 1..2178: mol_type = other RNA
gctgggattacaggcatgagccactgtgcccggccaactttctacaagaagaacatccacatacctcaagcaattcttacgccaccctgtaaagttctacagggacagtattagttgctccattttacagatgagaacactaaagcttggagaggccgagccacttgcccaaggtgatatggttgtttatcggcagatggagtgggaactgaaacgaggtctttggagtctgactgcagctcccaacactgccccacgcagctcaccctgtgcagatgggaccccgggcaatactgctccaacgtcatcatcctgtccagtaaacctttcttttgagatccaggccattcctctcttgcactccttttctccctgctcagctggcagtctgtcctgagctgacttacccataggaggacactcagagaggaaccctagggagggggtcatctcatccccttatttttggatgaagaaacagaggcctgagaggagaggagactgatcccaatctctcctggtgtccagcctgtgcccgtccactacccccgctgcttcttttaaggaacggagcctcactggtgccagcaggtgcaccacaccacctgcctcgcccctaccttgccgatgacgtcattgcggctgagcttgtccttgtccatgacagtgatgatgatggtcgtctccctcagcttctccgtggggatatcgaaggcgaaggactcattgaagatggggttcaggttcctcttcatcgtcaccgtcttcttcttctccacccgcttgtccttgtacatcagccataccttcacgtaggggtctgatgtgcccccgatgtccatggctttgaggttccgggctttgatgatgttcacgatgatggagttggcagaggggttgtagcagagagacaagagcagctcccctcggctcccactcccatcgctgcatggcttcagatccttccagaaggtctgcatctgggtcaggtccaccttgttaagggggatggacacctccccaatggggtcgttgcggctgaagcggtcatagtccaggacttggaggtagaggatcctctgcaccaccttctcatagggaaaaccttcaaagaggaaggtctcgttccagtgggggttcaggttcttccgcttcaccttggtctccagcttgtgcttcttgtcgggcagcaggtagatcttgacgaaggggtcgctggtgccgctgaagtccttggccggcagctcctgggccttcatgatcttcacggtgagcgtggactcctggaagttgtagccgacactgaactggatccggcccaggttctctcggctgcaaccctcgtgggcctcatcctcctcggagcctggggagagcatgagcatctcgctggtgagggagttgacgaggtctgagacggaggaacgtggctcggtccggcggtcggactcatcgtggggtgtctggcctggcacgggggctgtgttcaccgccttccctcctgcaggcaacaggaaggatttcatgtccaagcctcggtttcgaatctgccccaccacgtggtcccagctgcctgggttggagcggctgcggccccctgccgcccggtacttggagccggccgaggtgccctgccgagcctggccccggccataggcccgggggttggggcctggtgccgaggccatgtgggcctgcagctggcccaggctctggctggtggtgggctggctgggctgccggccccgctggtgctggctcagcggctgttgcaggctctgctgccgcatcagggtgcggggtcgctggcatttcggctctcccgtggagctggggatagactcaagggtagtggccgtggacagggtggagtcctcgaaacttggggcaggtggaggagaggagagaaaggagaagcagatgaagggatcacagtggaagagaaagaagccgagggccaggactaggaggccccagtgcagggtgcgcgctgccggacctcgccaggcctccatcggagctgtcgccaccgccgtcgccgccactgcctcgcccaggaggctgcaaagccctcgcgcccaccctgaggccccaggccggctctgcccacccaccttctggccctggctcagctagtgccagaatacctcctggctaggccgacctccctgccggtct

SEQ ID NO: 15679 - RNA, 1983 nt, Homo sapiens
  source 1..1983: mol_type = other RNA
gctgggattacaggcatgagccactgtgcccggccaactttctacaagaagaacatccacatacctcaagcaattcttacgccaccctgtaaagttctacagggacagtattagttgctccattttacagatgagaacactaaagcttggagaggccgagccacttgcccaaggtgatatggttgtttatcggcagatggagtgggaactgaaacgaggtctttggagtctgactgcagctcccaacactgccccacgcagctcaccctgtgcagatgggaccccgggcaatactgctccaacgtcatcatcctgtccagtaaacctttcttttgagatccaggccattcctctcttgcactccttttctccctgctcagctggcagtctgtcctgagctgacttacccataggaggacactcagagaggaaccctagggagggggtcatctcatccccttatttttggatgaagaaacagaggcctgagaggagaggagactgatcccaatctctcctggtgtccagcctgtgcccgtccactacccccgctgcttcttttaaggaacggagcctcactggtgccagcaggtgcaccacaccacctgcctcgcccctaccttgccgatgacgtcattgcggctgagcttgtccttgtccatgacagtgatgatgatggtcgtctccctcagcttctccgtggggatatcgaaggcgaaggactcattgaagatggggttcaggttcctcttcatcgtcaccgtcttcttcttctccacccgcttgtccttgtacatcagccataccttcacgtaggggtctgatgtgcccccgatgtccatggctttgaggttccgggctttgatgatgttcacgatgatggagttggcagaggggttgtagcagagagacaagagcagctcccctcggctcccactcccatcgctgcatggcttcagatccttccagaaggtctgcatctgggtcaggtccaccttgttaagggggatggacacctccccaatggggtcgttgcggctgaagcggtcatagtccaggacttggaggtagaggatcctctgcaccaccttctcatagggaaaaccttcaaagaggaaggtctcgttccagtgggggttcaggttcttccgcttcaccttggtctccagcttgtgcttcttgtcgggcagcaggtagatcttgacgaaggggtcgctggtgccgctgaagtccttggccggcagctcctgggccttcatgatcttcacggtgagcgtggactcctggaagttgtagccgacactgaactggatccggcccaggttctctcggctgcaaccctcgtgggcctcatcctcctcggagcctggggagagcatgagcatctcgctggtgagggagttgacgaggtctgagacggaggaacgtggctcggtccggcggtcggactcatcgtggggtgtctggcctggcacgggggctgtgttcaccgccttccctcctgcaggcaacttgatagccttcttctcactgcgcccacgccctgagtctggcgtgcccaccgtctccaaggaattcttgtagcgtttgcccagtttgcgctgacaccagtggcagaggccgcagaggacgacagtgacgctaaggctgacggtgatgatggcagagaccagcaggacgtcgcgcgagggcgcccctgggctggccgcctccgggtcccggtacatggtcccctcgtcgccggttccctccgggctcctcagagccgcccgcggccgcgcgctgctccgccgccgccgctgggcatggggccgggcgacccccgggggcgggtccgagggcgggggccgagcgggctgcacctagccgcggagccggggagcgggggccgcccgccagccctcccgcccgcccgcggagcacgctgccgccgccgccgaacagcgccgagccgcctccctccggcctgcgcgccgcgtgtgc

SEQ ID NO: 15680 - RNA, 3038 nt, Homo sapiens
  source 1..3038: mol_type = other RNA
gctgggattacaggcatgagccactgtgcccggccaataataggtaatacttttattatatgtagtcactgtttgaaacacttctacaaataatgcatttaatccccaacacaaacctatgaggtagattaactgtcatcctcattttacagataaggaaactagtgcagtttttgtaacttaaccaaggacaaacacctggactcaaaccaaagtctgcctggctctgtattattaatcactactctctgcttcctgcaaaatcaagctggctgccagaggggatgctaaaacctaacacatttacatcttccctcatttccacaggtaacagcaataatggtaggttcttccatgatcataaaaaataactagatggaattgcaagaaaatgctgcctgctttgaggtcacttgaaacagcaatgagaataaatttaagacaaatggtgccttgcacctgactcaaagagtatatacatcctgacttttgcaaaggcacagagtacaactgtctagtgaagacaaactgaagaataagtagggtgggtggacactgaacctgagataggtctctggaagtttgcaccctactaggaatgtcttccaagatgcatttggctccacatggacagggcccgtttttgaatttaggagacttctgacgtacggactgcaatagggaatccatatatctgtctttttatttactggtttactccttgtgtagtgttgcacatatgagaaaggatgcatgggagataaagatttcagatttaaagggtctgaaatgcctttattctatacttatactttggagtatagaattgcaggggaaaacattttccatgagaagtctgaaggcatacacattgtcatctgactttgaaggttgctcttgaaaaatctaatgccattttcattttttactgtttttgagacaaagtctcactctgtcgcccaggctggagtgcagtggtgcgatctcagctcactgcaacctctgcctcagggattcaagtgattctcctgcctcagcctctctagtagctgggattacaggcatgcgccaccatgcctggctaatttttgtgtttttttttttcaggagagacggggtttcaccatattgggcgggctggtctcgaactcctgacctcatgatccacccgcctcagcctcccaaagtgctgggattacaggcacgagccaccgcgcctggccccgctttcatttctgatcttttgttttctctctctagaaactttttagggtctcattttttctccatgatcctcttattcaaacttggtgttttcataattcacagcaattttccttaatgtaggtttcccttgaatccatcctgctgggcacccagcatgtcctttaaatctggaaacttacatttccttttatgtttctaagtttgtttgtttgttttttggtcttctctaaccataaagagacttcatgttggggaaacaggttcaaaaaacttaaagaagagttcatgatgaaagccaagtgtctaaccaggaaggacagcgaggacactgataaaaagcatgaaaataaagagaaaaaaggagaggcacagtgggcctaactatggatagccctatgcttggacaggtgtcttctgagtgtgtagtttctgatgcagaatgaatcttccacaccagctgaaggttttaccacacactttacactcataaggtttctcgccagtgtgaactcgctggtgctgaatcagggttattttctgattgaatgccttcccacactccttacattcaaagggcttctccccagtgtgaattcgctgatgctgagtcaaggctgtgttggagcttaatcgttttccacactctttacattcataaggtttctccccagtgtgcattcgctgatggacagtgaaacttgagctgcaactgaaagttttccaacattcgttacattcatagagcttctccccagtgtggaacctctggtgctggaggaagacagagctgctactgaaggccttgccgcactccttacattcatagggcttttctccagtgtggattctctgatgctgaatcaaggctgtgtctgaacttaaaccttttccacattctttacatttaaatggtttctttccagtgtgaattatctgatgccgaataagtaatgagttatatctgaagtattttccacattctttgcattcaaaagacttttcaccagtgtgacatttctcatgtcggtggaagtctgccatttgaatgaaatatctgccacattgtccacattcataagatatctgaccactaggatttgtctgatttgtagtgagttgtgtgctgacgctaatattttttcctaatttctcaaacttctctccattcttgacctcataggcctcatggtgcctggctgaggtatctgtgaaatgtctcctctttgactttgtcttaattatccaatgaccttgtggctgctctaggctgctcccaaagtcaaggtgctgggaaacattccctggcaggccccccaccatcagtctgaaggactctgtttctttggacacatgatcctttggagttaatccttccttctcagttctggcctcatcccctggacagatacctctgagagcctccctgcccataggttcccagggatcgaggccccatggcagttccccttgctccagctgggagaccagaacaggcgtggtgaatgggaatgccagggaagccacatttgcataattctccagcatcacttccctgtacagggccctctgcacagagtccaggctggcccattcattctgggtgaagtacacagccacatcctcaaaggtcactggttcctggcgccaagcggtctggaacatggctggcgtcccagcttcacacactgcctcagggttcggagaagtgaaaccggaccgcgaacctcttcagctcggaccgcgaatcccgcgcggcgcaggcgcagataaagcgtggaaattccacctgccgccgacaccggggaaagctt

SEQ ID NO: 15681 - RNA, 2859 nt, Homo sapiens
  source 1..2859: mol_type = other RNA
gctgggattacaggcatgagccactgtgcccggccaataataggtaatacttttattatatgtagtcactgtttgaaacacttctacaaataatgcatttaatccccaacacaaacctatgaggtagattaactgtcatcctcattttacagataaggaaactagtgcagtttttgtaacttaaccaaggacaaacacctggactcaaaccaaagtctgcctggctctgtattattaatcactactctctgcttcctgcaaaatcaagctggctgccagaggggatgctaaaacctaacacatttacatcttccctcatttccacaggtaacagcaataatggtaggttcttccatgatcataaaaaataactagatggaattgcaagaaaatgctgcctgctttgaggtcacttgaaacagcaatgagaataaatttaagacaaatggtgccttgcacctgactcaaagagtatatacatcctgacttttgcaaaggcacagagtacaactgtctagtgaagacaaactgaagaataagtagggtgggtggacactgaacctgagataggtctctggaagtttgcaccctactaggaatgtcttccaagatgcatttggctccacatggacagggcccgtttttgaatttaggagacttctgacgtacggactgcaatagggaatccatatatctgtctttttatttactggtttactccttgtgtagtgttgcacatatgagaaaggatgcatgggagataaagatttcagatttaaagggtctgaaatgcctttattctatacttatactttggagtatagaattgcaggggaaaacattttccatgagaagtctgaaggcatacacattgtcatctgactttgaaggttgctcttgaaaaatctaatgccattttcattttttactgtttttgagacaaagtctcactctgtcgcccaggctggagtgcagtggtgcgatctcagctcactgcaacctctgcctcagggattcaagtgattctcctgcctcagcctctctagtagctgggattacaggcatgcgccaccatgcctggctaatttttgtgtttttttttttcaggagagacggggtttcaccatattgggcgggctggtctcgaactcctgacctcatgatccacccgcctcagcctcccaaagtgctgggattacaggcacgagccaccgcgcctggccccgctttcatttctgatcttttgttttctctctctagaaactttttagggtctcattttttctccatgatcctcttattcaaacttggtgttttcataattcacagcaattttccttaatgtaggtttcccttgaatccatcctgctgggcacccagcatgtcctttaaatctggaaacttacatttccttttatgtttctaagtttgtttgtttgttttttggtcttctctaaccataaagagacttcatgttggggaaacaggttcaaaaaacttaaagaagagttcatgatgaaagccaagtgtctaaccaggaaggacagcgaggacactgataaaaagcatgaaaataaagagaaaaaaggagaggcacagtgggcctaactatggatagccctatgcttggacaggtgtcttctgagtgtgtagtttctgatgcagaatgaatcttccacaccagctgaaggttttaccacacactttacactcataaggtttctcgccagtgtgaactcgctggtgctgaatcagggttattttctgattgaatgccttcccacactccttacattcaaagggcttctccccagtgtgaattcgctgatgctgagtcaaggctgtgttggagcttaatcgttttccacactctttacattcataaggtttctccccagtgtgcattcgctgatggacagtgaaacttgagctgcaactgaaagttttccaacattcgttacattcatagagcttctccccagtgtggaacctctggtgctggaggaagacagagctgctactgaaggccttgccgcactccttacattcatagggcttttctccagtgtggattctctgatgctgaatcaaggctgtgtctgaacttaaaccttttccacattctttacatttaaatggtttctttccagtgtgaattatctgatgccgaataagtaatgagttatatctgaagtattttccacattctttgcattcaaaagacttttcaccagtgtgacatttctcatgtcggtggaagtctgccatttgaatgaaatatctgccacattgtccacattcataagatatctgaccactaggatttgtctgatttgtagtgagttgtgtgctgacgctaatattttttcctaatttctcaaacttctctccattcttgacctcataggcctcatggtgcctggctgaggtatctgtgaaatgtctcctctttgactttgtcttaattatccaatgaccttgtggctgctctaggctgctcccaaagtcaaggtgctgggaaacattccctggcaggccccccaccatcagtctgaaggactctgtttctttggacacatgatcctttggagttaatccttccttctcagttctggcctcatcccctggcgccaagcggtctggaacatggctggcgtcccagcttcacacactgcctcagggttcggagaagtgaaacccaaaaagcaaaggggttgcaaaaccaggcagaacaagccccaggaaaaccaatcagttacccggaccgcgaacctcttcagctcggaccgcgaatcccgcgcggcgcaggcgcagataaagcgtggaaattccacctgccgccgacaccggggaaagctt

SEQ ID NO: 15682 - RNA, 2797 nt, Homo sapiens
  source 1..2797: mol_type = other RNA
gctgggattacaggcatgagccactgtgcccggccaataataggtaatacttttattatatgtagtcactgtttgaaacacttctacaaataatgcatttaatccccaacacaaacctatgaggtagattaactgtcatcctcattttacagataaggaaactagtgcagtttttgtaacttaaccaaggacaaacacctggactcaaaccaaagtctgcctggctctgtattattaatcactactctctgcttcctgcaaaatcaagctggctgccagaggggatgctaaaacctaacacatttacatcttccctcatttccacaggtaacagcaataatggtaggttcttccatgatcataaaaaataactagatggaattgcaagaaaatgctgcctgctttgaggtcacttgaaacagcaatgagaataaatttaagacaaatggtgccttgcacctgactcaaagagtatatacatcctgacttttgcaaaggcacagagtacaactgtctagtgaagacaaactgaagaataagtagggtgggtggacactgaacctgagataggtctctggaagtttgcaccctactaggaatgtcttccaagatgcatttggctccacatggacagggcccgtttttgaatttaggagacttctgacgtacggactgcaatagggaatccatatatctgtctttttatttactggtttactccttgtgtagtgttgcacatatgagaaaggatgcatgggagataaagatttcagatttaaagggtctgaaatgcctttattctatacttatactttggagtatagaattgcaggggaaaacattttccatgagaagtctgaaggcatacacattgtcatctgactttgaaggttgctcttgaaaaatctaatgccattttcattttttactgtttttgagacaaagtctcactctgtcgcccaggctggagtgcagtggtgcgatctcagctcactgcaacctctgcctcagggattcaagtgattctcctgcctcagcctctctagtagctgggattacaggcatgcgccaccatgcctggctaatttttgtgtttttttttttcaggagagacggggtttcaccatattgggcgggctggtctcgaactcctgacctcatgatccacccgcctcagcctcccaaagtgctgggattacaggcacgagccaccgcgcctggccccgctttcatttctgatcttttgttttctctctctagaaactttttagggtctcattttttctccatgatcctcttattcaaacttggtgttttcataattcacagcaattttccttaatgtaggtttcccttgaatccatcctgctgggcacccagcatgtcctttaaatctggaaacttacatttccttttatgtttctaagtttgtttgtttgttttttggtcttctctaaccataaagagacttcatgttggggaaacaggttcaaaaaacttaaagaagagttcatgatgaaagccaagtgtctaaccaggaaggacagcgaggacactgataaaaagcatgaaaataaagagaaaaaaggagaggcacagtgggcctaactatggatagccctatgcttggacaggtgtcttctgagtgtgtagtttctgatgcagaatgaatcttccacaccagctgaaggttttaccacacactttacactcataaggtttctcgccagtgtgaactcgctggtgctgaatcagggttattttctgattgaatgccttcccacactccttacattcaaagggcttctccccagtgtgaattcgctgatgctgagtcaaggctgtgttggagcttaatcgttttccacactctttacattcataaggtttctccccagtgtgcattcgctgatggacagtgaaacttgagctgcaactgaaagttttccaacattcgttacattcatagagcttctccccagtgtggaacctctggtgctggaggaagacagagctgctactgaaggccttgccgcactccttacattcatagggcttttctccagtgtggattctctgatgctgaatcaaggctgtgtctgaacttaaaccttttccacattctttacatttaaatggtttctttccagtgtgaattatctgatgccgaataagtaatgagttatatctgaagtattttccacattctttgcattcaaaagacttttcaccagtgtgacatttctcatgtcggtggaagtctgccatttgaatgaaatatctgccacattgtccacattcataagatatctgaccactaggatttgtctgatttgtagtgagttgtgtgctgacgctaatattttttcctaatttctcaaacttctctccattcttgacctcataggcctcatggtgcctggctgaggtatctgtgaaatgtctcctctttgactttgtcttaattatccaatgaccttgtggctgctctaggctgctcccaaagtcaaggtgctgggaaacattccctggcaggccccccaccatcagtctgaaggactctgtttctttggacacatgatcctttggagttaatccttccttctcagttctggcctcatcccctggcgccaagcggtctggaacatggctggcgtcccagcttcacacactgcctcagggttcggagaagtgaaaccggaccgcgaacctcttcagctcggaccgcgaatcccgcgcggcgcaggcgcagataaagcgtggaaattccacctgccgccgacaccggggaaagctt

SEQ ID NO: 15683 - RNA, 3560 nt, Homo sapiens
  source 1..3560: mol_type = other RNA
gctgggattacaggcatgagccactgtgcccggccagaaagatgattgtaaaaatggactgggtggtctgaaggaagggcaaggaagacccatttgctggttttgttaaagaaaaaaaaaaaagtacatataatgcctggatttgcctttgggagggaaatcctgcccagtccctctttcttccaggcatggaatcctaggctgtgggataatgagcacaatgccaagtgtcagctggacagagaggaagggcatgagggatgggctttggtgcacatgacgctggggacagtagaggacagaggaggaactacacatgtggggcccctacccttgagctgcacccagattttcatcaagggcccatcaggatcaggtgtctgtgggagcctcttgcctagggtgagcttagactgcatcacaccttcaacagttcccctgcaactctcaaataatggataggttaaagccagaggagggttaatttgcccacaagtctttctgtgctttccttgtgccatcactcagctaggcagaatacattctctcgctcttagccatcccaagggaggcagagatgatcagacataacttttgaacccccatctcactggagaagggaaatcctacatgggaaatgctcatcctgcccaacttggggctggcaccttcatttccaaatgatgctggggagtcaggtcagtttctgtactggaagcataaagcacatggcttgaaatcagctcccaggaaaggatcattctttgtgcctgagagcaaagccaagggaaacgtggcaaaaagaggtcactttgttaatattccccttctctccaccaatccccttattcagaatgcagcaaggcagttttctagtcatgcagtccacgcatgaggaataaatacacctcatgtcttccacctgctgccagtgcggtgatgagatgcagagctgaggggctgaggaagaggcttctgtgtcaaggtagattcagctggtggtctagtattgcccaaacgacttccgtagggataggaaaggcccctgcttgttaacaaagaagagggaaagggcagagaacctggatccatctgagatctgtgggctttttactttttcagccatttgagggttgactggctctaaggaaaagctgtttgctggcagacacaggtggctggtgacaaagggaacagagcaggggaatggatagctcaaaacgagcctcgccactcctgaacagaacagcaatcccagctgtgtcctttcgagggtgagtgaaagcacatgctgtcctttacatgcttgaggcggacttgcctgtctcttcaggccggatgctcttcagggccctgtggggcttaaacacatgtactgagctagctccaatcttaatctgcacaacatcgcaacccctgagttcctattagttcttggtcccagtgtggatcgctctgagagaccacagctccctcctctggagtcccctctccgagctctccaagggaaaagacaaaggaagccgaactgccaagttgaagattttgcctcaggcaaaagttcttcgtgaccaggtgggtcttgtaatgcttggtgaggtggtcactcctcatgaagcgcttctgacactgggcgcactcgaagcgtttgtcccctgtgtgggtgcgagcatgccgttggagctcgtcactccgtgtgaacctcttcccacagaagaaccagttgcagacaaagggccgctcgccagtgtgcaggcgcacatgggcacgcagcaaggacgtcttacggaacgtcttgccacagtcggggatgtggcacacgtgcttcttcttgccctgctctccagacctcttctccccatccttgcagttgggacacgtgcaggccatgcggcgccgcttctccccgggctgggtctctccggccagggcttgttccatttgcagctggatctgggtggggctcagcccactgatggtcaggttgttcccagaaacattctgcactgtcagctgctgctgcccgcctgtgttggtgatggtgacaggcacgccctggacctggacaccattgatgttgatggtctgcattgcctgggcagctgccgccaactgggctgcattcaggctgatgatgctcccggctggggcaatctttggcaggggacgctcttttcggagaattgcagctgagtgctttttgctggtcccactcagatggggagcacgggatgcagggctgctacaggtggtgttagaggtggctgcagctgttgctggggggctgtcctggacaaggactgtctgcacctcaccggaaggcgtgcggatgtagacctgagtaggtgtcggctcagctgcctggatctgaaagttctgggagggcttctggggtacagtggggagggtggcagatgccgcctgcaccacccgcagagcctgctgggggatctgtaccacctgctgctgctcggccttggggggcaccacctggacctgctggaccacagctggctggcccccaccagggctctgaacaatgagcaggttatttcctgcctggatgatgttgtccgcggtggtctcgatcagcaccgtctccacctgctcagccacagccacagggggctgggaggcaggaaggctcttcttccttgctttcttgttagtcttagacagcggggttggggggctttcagtgaggagctgagtaggggccccggtgtcactggcgttcacaaggttgttgacgggcagagtgagcgtcacattgccgcccccacctgtcagcttcaccacattggccccgctctgcacgggggtggtggtcgtactcgacttctggatgggggctggcttgatggggacaggcttgtgactggacggtgagggggtgatgatggcttggttggtgccagggatgatctggatctggttggtgagattgggctgtacttggatggtttgggaattgcttgcctgaatctgagggaccgcctggtactggatattggcatttgatcgggtccctttgttgatcatggtgggattctggatagcgaacaccagctgccctccaggataggaggcgctcagttgtgacccctgaatctgaagtatatttcctttggaggacaagattccaaagctattcttgccggggctgagagggagaggggcaggtttgatagggacaagtttccgcggtgtgggctgtgggggagcaggaggtgtcacagcagcttcaactgctggagggccaattttgctacatgttgcagcaagcagggctaagggagatggctgggagtcctgggtggtggaggcggcaggctgcaggtagtcactgggactcacagcagcagtggcagccatgctggtctgtggatatctatttcagtagattactttctcctctcctctcctcagactcagccatctgaggctgtgaggacagctggtcctgctgtcgttggactgccccctccagccaccacagagtcgctcattacgacatcttcctccctggcctccgccgcctccgccgccaccgagagcct

SEQ ID NO: 15684 - RNA, 3614 nt, Homo sapiens
  source 1..3614: mol_type = other RNA
gctgggattacaggcatgagccactgtgcccggccagaaagatgattgtaaaaatggactgggtggtctgaaggaagggcaaggaagacccatttgctggttttgttaaagaaaaaaaaaaaagtacatataatgcctggatttgcctttgggagggaaatcctgcccagtccctctttcttccaggcatggaatcctaggctgtgggataatgagcacaatgccaagtgtcagctggacagagaggaagggcatgagggatgggctttggtgcacatgacgctggggacagtagaggacagaggaggaactacacatgtggggcccctacccttgagctgcacccagattttcatcaagggcccatcaggatcaggtgtctgtgggagcctcttgcctagggtgagcttagactgcatcacaccttcaacagttcccctgcaactctcaaataatggataggttaaagccagaggagggttaatttgcccacaagtctttctgtgctttccttgtgccatcactcagctaggcagaatacattctctcgctcttagccatcccaagggaggcagagatgatcagacataacttttgaacccccatctcactggagaagggaaatcctacatgggaaatgctcatcctgcccaacttggggctggcaccttcatttccaaatgatgctggggagtcaggtcagtttctgtactggaagcataaagcacatggcttgaaatcagctcccaggaaaggatcattctttgtgcctgagagcaaagccaagggaaacgtggcaaaaagaggtcactttgttaatattccccttctctccaccaatccccttattcagaatgcagcaaggcagttttctagtcatgcagtccacgcatgaggaataaatacacctcatgtcttccacctgctgccagtgcggtgatgagatgcagagctgaggggctgaggaagaggcttctgtgtcaaggtagattcagctggtggtctagtattgcccaaacgacttccgtagggataggaaaggcccctgcttgttaacaaagaagagggaaagggcagagaacctggatccatctgagatctgtgggctttttactttttcagccatttgagggttgactggctctaaggaaaagctgtttgctggcagacacaggtggctggtgacaaagggaacagagcaggggaatggatagctcaaaacgagcctcgccactcctgaacagaacagcaatcccagctgtgtcctttcgagggtgagtgaaagcacatgctgtcctttacatgcttgaggcggacttgcctgtctcttcaggccggatgctcttcagggccctgtggggcttaaacacatgtactgagctagctccaatcttaatctgcacaacatcgcaacccctgagttcctattagttcttggtcccagtgtggatcgctctgagagaccacagctccctcctctggagtcccctctccgagctctccaagggaaaagacaaaggaagccgaactgccaagttgaagattttgcctcaggcaaaagttcttcgtgaccaggtgggtcttgtaatgcttggtgaggtggtcactcctcatgaagcgcttctgacactgggcgcactcgaagcgtttgtcccctgtgtgggtgcgagcatgccgttggagctcgtcactccgtgtgaacctcttcccacagaagaaccagttgcagacaaagggccgctcgccagtgtgcaggcgcacatgggcacgcagcaaggacgtcttacggaacgtcttgccacagtcggggatgtggcacacgtgcttcttcttgccctgctctccagacctcttctccccatccttgcagttgggacacgtgcaggccatgcggcgccgcttctccccgggctgggtctctccggccagggcttgttccatttgcagctggatctgggtggggctcagcccactgatggtcaggttgttcccagaaacattctgcactgtcagctgctgctgcccgcctgtgttggtgatggtgacaggcacgccctggacctggacaccattgatgttgatggtctgcattgcctgggcagctgccgccaactgggctgcattcaggctgatgatgctcccggctggggcaatctttggcaggggacgctcttttcggagaattgcagctgagtgctttttgctggtcccactcagatggggagcacgggatgcagggctgctacaggtggtgttagaggtggctgcagctgttgctggggggctgtcctggacaaggactgtctgcacctcaccggaaggcgtgcggatgtagacctgagtaggtgtcggctcagctgcctggatctgaaagttctgggagggcttctggggtacagtggggagggtggcagatgccgcctgcaccacccgcagagcctgctgggggatctgtaccacctgctgctgctcggccttggggggcaccacctggacctgctggaccacagctggctggcccccaccagggctctgaacaatgagcaggttatttcctgcctggatgatgttgtccgcggtggtctcgatcagcaccgtctccacctgctcagccacagccacagggggctgggaggcaggaaggctcttcttccttgctttcttgttagtcttagacagcggggttggggggctttcagtgaggagctgagtaggggccccggtgtcactggcgttcacaaggttgttgacgggcagagtgagcgtcacattgccgcccccacctgtcagcttcaccacattggccccgctctgcacgggggtggtggtcgtactcgacttctggatgggggctggcttgatggggacaggcttgtgactggacggtgagggggtgatgatggcttggttggtgccagggatgatctggatctggttggtgagattgggctgtacttggatggtttgggaattgcttgcctgaatctgagggaccgcctggtactggatattggcatttgatcgggtccctttgttgatcatggtgggattctggatagcgaacaccagctgccctccaggataggaggcgctcagttgtgacccctgaatctgaagtatatttcctttggaggacaagattccaaagctattcttgccggggctgagagggagaggggcaggtttgatagggacaagtttccgcggtgtgggctgtgggggagcaggaggtgtcacagcagcttcaactgctggagggccaattttgctacatgttgcagcaagcagggctaagggagatggctgggagtcctgggtggtggaggcggcaggctgcaggtagtcactgggactcacagcagcagtggcagccatgctggtctgtggatcaatcgtcccagccaatgataatccatttccaacaggtattaacgcctgttagaagccactggaacactgacatcatcagcccaattgataggttgtctgatagattcgcccccgctcattacgacatcttcctccctggcctccgccgcctccgccgccaccgagagcctgacaccgcccgccaagcaaccgccaatcccggagcccgccaccgcccgagcgac

SEQ ID NO: 15685 - RNA, 3660 nt, Homo sapiens
  source 1..3660: mol_type = other RNA
gctgggattacaggcatgagccactgtgcccggccagaaagatgattgtaaaaatggactgggtggtctgaaggaagggcaaggaagacccatttgctggttttgttaaagaaaaaaaaaaaagtacatataatgcctggatttgcctttgggagggaaatcctgcccagtccctctttcttccaggcatggaatcctaggctgtgggataatgagcacaatgccaagtgtcagctggacagagaggaagggcatgagggatgggctttggtgcacatgacgctggggacagtagaggacagaggaggaactacacatgtggggcccctacccttgagctgcacccagattttcatcaagggcccatcaggatcaggtgtctgtgggagcctcttgcctagggtgagcttagactgcatcacaccttcaacagttcccctgcaactctcaaataatggataggttaaagccagaggagggttaatttgcccacaagtctttctgtgctttccttgtgccatcactcagctaggcagaatacattctctcgctcttagccatcccaagggaggcagagatgatcagacataacttttgaacccccatctcactggagaagggaaatcctacatgggaaatgctcatcctgcccaacttggggctggcaccttcatttccaaatgatgctggggagtcaggtcagtttctgtactggaagcataaagcacatggcttgaaatcagctcccaggaaaggatcattctttgtgcctgagagcaaagccaagggaaacgtggcaaaaagaggtcactttgttaatattccccttctctccaccaatccccttattcagaatgcagcaaggcagttttctagtcatgcagtccacgcatgaggaataaatacacctcatgtcttccacctgctgccagtgcggtgatgagatgcagagctgaggggctgaggaagaggcttctgtgtcaaggtagattcagctggtggtctagtattgcccaaacgacttccgtagggataggaaaggcccctgcttgttaacaaagaagagggaaagggcagagaacctggatccatctgagatctgtgggctttttactttttcagccatttgagggttgactggctctaaggaaaagctgtttgctggcagacacaggtggctggtgacaaagggaacagagcaggggaatggatagctcaaaacgagcctcgccactcctgaacagaacagcaatcccagctgtgtcctttcgagggtgagtgaaagcacatgctgtcctttacatgcttgaggcggacttgcctgtctcttcaggccggatgctcttcagggccctgtggggcttaaacacatgtactgagctagctccaatcttaatctgcacaacatcgcaacccctgagttcctattagttcttggtcccagtgtggatcgctctgagagaccacagctccctcctctggagtcccctctccgagctctccaagggaaaagacaaaggaagccgaactgccaagttgaagattttgcctcaggcaaaagttcttcgtgaccaggtgggtcttgtaatgcttggtgaggtggtcactcctcatgaagcgcttctgacactgggcgcactcgaagcgtttgtcccctgtgtgggtgcgagcatgccgttggagctcgtcactccgtgtgaacctcttcccacagaagaaccagttgcagacaaagggccgctcgccagtgtgcaggcgcacatgggcacgcagcaaggacgtcttacggaacgtcttgccacagtcggggatgtggcacacgtgcttcttcttgccctgctctccagacctcttctccccatccttgcagttgggacacgtgcaggccatgcggcgccgcttctccccgggctgggtctctccggccagggcttgttccatttgcagctggatctgggtggggctcagcccactgatggtcaggttgttcccagaaacattctgcactgtcagctgctgctgcccgcctgtgttggtgatggtgacaggcacgccctggacctggacaccattgatgttgatggtctgcattgcctgggcagctgccgccaactgggctgcattcaggctgatgatgctcccggctggggcaatctttggcaggggacgctcttttcggagaattgcagctgagtgctttttgctggtcccactcagatggggagcacgggatgcagggctgctacaggtggtgttagaggtggctgcagctgttgctggggggctgtcctggacaaggactgtctgcacctcaccggaaggcgtgcggatgtagacctgagtaggtgtcggctcagctgcctggatctgaaagttctgggagggcttctggggtacagtggggagggtggcagatgccgcctgcaccacccgcagagcctgctgggggatctgtaccacctgctgctgctcggccttggggggcaccacctggacctgctggaccacagctggctggcccccaccagggctctgaacaatgagcaggttatttcctgcctggatgatgttgtccgcggtggtctcgatcagcaccgtctccacctgctcagccacagccacagggggctgggaggcaggaaggctcttcttccttgctttcttgttagtcttagacagcggggttggggggctttcagtgaggagctgagtaggggccccggtgtcactggcgttcacaaggttgttgacgggcagagtgagcgtcacattgccgcccccacctgtcagcttcaccacattggccccgctctgcacgggggtggtggtcgtactcgacttctggatgggggctggcttgatggggacaggcttgtgactggacggtgagggggtgatgatggcttggttggtgccagggatgatctggatctggttggtgagattgggctgtacttggatggtttgggaattgcttgcctgaatctgagggaccgcctggtactggatattggcatttgatcgggtccctttgttgatcatggtgggattctggatagcgaacaccagctgccctccaggataggaggcgctcagttgtgacccctgaatctgaagtatatttcctttggaggacaagattccaaagctattcttgccggggctgagagggagaggggcaggtttgatagggacaagtttccgcggtgtgggctgtgggggagcaggaggtgtcacagcagcttcaactgctggagggccaattttgctacatgttgcagcaagcagggctaagggagatggctgggagtcctgggtggtggaggcggcaggctgcaggtagtcactgggactcacagcagcagtggcagccatgctggtctgtggatcaatcgtcccagccaatgataatccatttccaacaggtattaacgcctgttagaagccactggaacactgacatcatcagcccaattgataggttgtctgatagattcgcccccgggctgtcgtcgatgccgagcagtgcccatctggttggcagcgtccgggtctcaagcgttccctcgcccctctctgttctccggggagccctgaatcgctggtgggcatcgctcattacgacatcttcctccctggcctccgccgcctccgccgcca

SEQ ID NO: 15686 - RNA, 3704 nt, Homo sapiens
  source 1..3704: mol_type = other RNA
gctgggattacaggcatgagccactgtgcccggccagaaagatgattgtaaaaatggactgggtggtctgaaggaagggcaaggaagacccatttgctggttttgttaaagaaaaaaaaaaaagtacatataatgcctggatttgcctttgggagggaaatcctgcccagtccctctttcttccaggcatggaatcctaggctgtgggataatgagcacaatgccaagtgtcagctggacagagaggaagggcatgagggatgggctttggtgcacatgacgctggggacagtagaggacagaggaggaactacacatgtggggcccctacccttgagctgcacccagattttcatcaagggcccatcaggatcaggtgtctgtgggagcctcttgcctagggtgagcttagactgcatcacaccttcaacagttcccctgcaactctcaaataatggataggttaaagccagaggagggttaatttgcccacaagtctttctgtgctttccttgtgccatcactcagctaggcagaatacattctctcgctcttagccatcccaagggaggcagagatgatcagacataacttttgaacccccatctcactggagaagggaaatcctacatgggaaatgctcatcctgcccaacttggggctggcaccttcatttccaaatgatgctggggagtcaggtcagtttctgtactggaagcataaagcacatggcttgaaatcagctcccaggaaaggatcattctttgtgcctgagagcaaagccaagggaaacgtggcaaaaagaggtcactttgttaatattccccttctctccaccaatccccttattcagaatgcagcaaggcagttttctagtcatgcagtccacgcatgaggaataaatacacctcatgtcttccacctgctgccagtgcggtgatgagatgcagagctgaggggctgaggaagaggcttctgtgtcaaggtagattcagctggtggtctagtattgcccaaacgacttccgtagggataggaaaggcccctgcttgttaacaaagaagagggaaagggcagagaacctggatccatctgagatctgtgggctttttactttttcagccatttgagggttgactggctctaaggaaaagctgtttgctggcagacacaggtggctggtgacaaagggaacagagcaggggaatggatagctcaaaacgagcctcgccactcctgaacagaacagcaatcccagctgtgtcctttcgagggtgagtgaaagcacatgctgtcctttacatgcttgaggcggacttgcctgtctcttcaggccggatgctcttcagggccctgtggggcttaaacacatgtactgagctagctccaatcttaatctgcacaacatcgcaacccctgagttcctattagttcttggtcccagtgtggatcgctctgagagaccacagctccctcctctggagtcccctctccgagctctccaagggaaaagacaaaggaagccgaactgccaagttgaagattttgcctcaggcaaaagttcttcgtgaccaggtgggtcttgtaatgcttggtgaggtggtcactcctcatgaagcgcttctgacactgggcgcactcgaagcgtttgtcccctgtgtgggtgcgagcatgccgttggagctcgtcactccgtgtgaacctcttcccacagaagaaccagttgcagacaaagggccgctcgccagtgtgcaggcgcacatgggcacgcagcaaggacgtcttacggaacgtcttgccacagtcggggatgtggcacacgtgcttcttcttgccctgctctccagacctcttctccccatccttgcagttgggacacgtgcaggccatgcggcgccgcttctccccgggctgggtctctccggccagggcttgttccatttgcagctggatctgggtggggctcagcccactgatggtcaggttgttcccagaaacattctgcactgtcagctgctgctgcccgcctgtgttggtgatggtgacaggcacgccctggacctggacaccattgatgttgatggtctgcattgcctgggcagctgccgccaactgggctgcattcaggctgatgatgctcccggctggggcaatctttggcaggggacgctcttttcggagaattgcagctgagtgctttttgctggtcccactcagatggggagcacgggatgcagggctgctacaggtggtgttagaggtggctgcagctgttgctggggggctgtcctggacaaggactgtctgcacctcaccggaaggcgtgcggatgtagacctgagtaggtgtcggctcagctgcctggatctgaaagttctgggagggcttctggggtacagtggggagggtggcagatgccgcctgcaccacccgcagagcctgctgggggatctgtaccacctgctgctgctcggccttggggggcaccacctggacctgctggaccacagctggctggcccccaccagggctctgaacaatgagcaggttatttcctgcctggatgatgttgtccgcggtggtctcgatcagcaccgtctccacctgctcagccacagccacagggggctgggaggcaggaaggctcttcttccttgctttcttgttagtcttagacagcggggttggggggctttcagtgaggagctgagtaggggccccggtgtcactggcgttcacaaggttgttgacgggcagagtgagcgtcacattgccgcccccacctgtcagcttcaccacattggccccgctctgcacgggggtggtggtcgtactcgacttctggatgggggctggcttgatggggacaggcttgtgactggacggtgagggggtgatgatggcttggttggtgccagggatgatctggatctggttggtgagattgggctgtacttggatggtttgggaattgcttgcctgaatctgagggaccgcctggtactggatattggcatttgatcgggtccctttgttgatcatggtgggattctggatagcgaacaccagctgccctccaggataggaggcgctcagttgtgacccctgaatctgaagtatatttcctttggaggacaagattccaaagctattcttgccggggctgagagggagaggggcaggtttgatagggacaagtttccgcggtgtgggctgtgggggagcaggaggtgtcacagcagcttcaactgctggagggccaattttgctacatgttgcagcaagcagggctaagggagatggctgggagtcctgggtggtggaggcggcaggctgcaggtagtcactgggactcacagcagcagtggcagccatgctggtctgtggatccaccctgggttgatagccttacatctatttcagtagattactttctcctctcctctcctcagactcagccatctgaggctgtgaggacagctggtcctgctgtcgttggactgccccctccagccaccacagagtcaatcgtcccagccaatgataatccatttccaacaggtattaacgcctgttagaagccactggaacactgacatcatcagcccaattgataggttgtctgatagattcgcccccgctcattacgacatcttcctccctggcctccgccgcctccgccgccaccgagagcctgacaccgc

SEQ ID NO: 15687 - RNA, 3695 nt, Homo sapiens
  source 1..3695: mol_type = other RNA
gctgggattacaggcatgagccactgtgcccggccagaaagatgattgtaaaaatggactgggtggtctgaaggaagggcaaggaagacccatttgctggttttgttaaagaaaaaaaaaaaagtacatataatgcctggatttgcctttgggagggaaatcctgcccagtccctctttcttccaggcatggaatcctaggctgtgggataatgagcacaatgccaagtgtcagctggacagagaggaagggcatgagggatgggctttggtgcacatgacgctggggacagtagaggacagaggaggaactacacatgtggggcccctacccttgagctgcacccagattttcatcaagggcccatcaggatcaggtgtctgtgggagcctcttgcctagggtgagcttagactgcatcacaccttcaacagttcccctgcaactctcaaataatggataggttaaagccagaggagggttaatttgcccacaagtctttctgtgctttccttgtgccatcactcagctaggcagaatacattctctcgctcttagccatcccaagggaggcagagatgatcagacataacttttgaacccccatctcactggagaagggaaatcctacatgggaaatgctcatcctgcccaacttggggctggcaccttcatttccaaatgatgctggggagtcaggtcagtttctgtactggaagcataaagcacatggcttgaaatcagctcccaggaaaggatcattctttgtgcctgagagcaaagccaagggaaacgtggcaaaaagaggtcactttgttaatattccccttctctccaccaatccccttattcagaatgcagcaaggcagttttctagtcatgcagtccacgcatgaggaataaatacacctcatgtcttccacctgctgccagtgcggtgatgagatgcagagctgaggggctgaggaagaggcttctgtgtcaaggtagattcagctggtggtctagtattgcccaaacgacttccgtagggataggaaaggcccctgcttgttaacaaagaagagggaaagggcagagaacctggatccatctgagatctgtgggctttttactttttcagccatttgagggttgactggctctaaggaaaagctgtttgctggcagacacaggtggctggtgacaaagggaacagagcaggggaatggatagctcaaaacgagcctcgccactcctgaacagaacagcaatcccagctgtgtcctttcgagggtgagtgaaagcacatgctgtcctttacatgcttgaggcggacttgcctgtctcttcaggccggatgctcttcagggccctgtggggcttaaacacatgtactgagctagctccaatcttaatctgcacaacatcgcaacccctgagttcctattagttcttggtcccagtgtggatcgctctgagagaccacagctccctcctctggagtcccctctccgagctctccaagggaaaagacaaaggaagccgaactgccaagttgaagattttgcctcaggcaaaagttcttcgtgaccaggtgggtcttgtaatgcttggtgaggtggtcactcctcatgaagcgcttctgacactgggcgcactcgaagcgtttgtcccctgtgtgggtgcgagcatgccgttggagctcgtcactccgtgtgaacctcttcccacagaagaaccagttgcagacaaagggccgctcgccagtgtgcaggcgcacatgggcacgcagcaaggacgtcttacggaacgtcttgccacagtcggggatgtggcacacgtgcttcttcttgccctgctctccagacctcttctccccatccttgcagttgggacacgtgcaggccatgcggcgccgcttctccccgggctgggtctctccggccagggcttgttccatttgcagctggatctgggtggggctcagcccactgatggtcaggttgttcccagaaacattctgcactgtcagctgctgctgcccgcctgtgttggtgatggtgacaggcacgccctggacctggacaccattgatgttgatggtctgcattgcctgggcagctgccgccaactgggctgcattcaggctgatgatgctcccggctggggcaatctttggcaggggacgctcttttcggagaattgcagctgagtgctttttgctggtcccactcagatggggagcacgggatgcagggctgctacaggtggtgttagaggtggctgcagctgttgctggggggctgtcctggacaaggactgtctgcacctcaccggaaggcgtgcggatgtagacctgagtaggtgtcggctcagctgcctggatctgaaagttctgggagggcttctggggtacagtggggagggtggcagatgccgcctgcaccacccgcagagcctgctgggggatctgtaccacctgctgctgctcggccttggggggcaccacctggacctgctggaccacagctggctggcccccaccagggctctgaacaatgagcaggttatttcctgcctggatgatgttgtccgcggtggtctcgatcagcaccgtctccacctgctcagccacagccacagggggctgggaggcaggaaggctcttcttccttgctttcttgttagtcttagacagcggggttggggggctttcagtgaggagctgagtaggggccccggtgtcactggcgttcacaaggttgttgacgggcagagtgagcgtcacattgccgcccccacctgtcagcttcaccacattggccccgctctgcacgggggtggtggtcgtactcgacttctggatgggggctggcttgatggggacaggcttgtgactggacggtgagggggtgatgatggcttggttggtgccagggatgatctggatctggttggtgagattgggctgtacttggatggtttgggaattgcttgcctgaatctgagggaccgcctggtactggatattggcatttgatcgggtccctttgttgatcatggtgggattctggatagcgaacaccagctgccctccaggataggaggcgctcagttgtgacccctgaatctgaagtatatttcctttggaggacaagattccaaagctattcttgccggggctgagagggagaggggcaggtttgatagggacaagtttccgcggtgtgggctgtgggggagcaggaggtgtcacagcagcttcaactgctggagggccaattttgctacatgttgcagcaagcagggctaagggagatggctgggagtcctgggtggtggaggcggcaggctgcaggtagtcactgggactcacagcagcagtggcagccatgctggtctgtggatccttgggggccgggaagaccccgccggcagcggccgggacccaccgctcattacgacatcttcctccctggcctccgccgcctccgccgccaccgagagcctgacaccgcccgccaagcaaccgccaatcccggagcccgccaccgcccgagcgacggcagccttcaccaataagcgcttggaacattggggaccgacagcactattaaccaatcaaccagaggcgtctagagcgacgttgatttgaccaataggtctgtgcaatgtcactgatggacggtagagcgcaccaaccgaaagccaatt

SEQ ID NO: 15688 - RNA, 3527 nt, Homo sapiens
  source 1..3527: mol_type = other RNA
gctgggattacaggcatgagccactgtgcccggccagaaagatgattgtaaaaatggactgggtggtctgaaggaagggcaaggaagacccatttgctggttttgttaaagaaaaaaaaaaaagtacatataatgcctggatttgcctttgggagggaaatcctgcccagtccctctttcttccaggcatggaatcctaggctgtgggataatgagcacaatgccaagtgtcagctggacagagaggaagggcatgagggatgggctttggtgcacatgacgctggggacagtagaggacagaggaggaactacacatgtggggcccctacccttgagctgcacccagattttcatcaagggcccatcaggatcaggtgtctgtgggagcctcttgcctagggtgagcttagactgcatcacaccttcaacagttcccctgcaactctcaaataatggataggttaaagccagaggagggttaatttgcccacaagtctttctgtgctttccttgtgccatcactcagctaggcagaatacattctctcgctcttagccatcccaagggaggcagagatgatcagacataacttttgaacccccatctcactggagaagggaaatcctacatgggaaatgctcatcctgcccaacttggggctggcaccttcatttccaaatgatgctggggagtcaggtcagtttctgtactggaagcataaagcacatggcttgaaatcagctcccaggaaaggatcattctttgtgcctgagagcaaagccaagggaaacgtggcaaaaagaggtcactttgttaatattccccttctctccaccaatccccttattcagaatgcagcaaggcagttttctagtcatgcagtccacgcatgaggaataaatacacctcatgtcttccacctgctgccagtgcggtgatgagatgcagagctgaggggctgaggaagaggcttctgtgtcaaggtagattcagctggtggtctagtattgcccaaacgacttccgtagggataggaaaggcccctgcttgttaacaaagaagagggaaagggcagagaacctggatccatctgagatctgtgggctttttactttttcagccatttgagggttgactggctctaaggaaaagctgtttgctggcagacacaggtggctggtgacaaagggaacagagcaggggaatggatagctcaaaacgagcctcgccactcctgaacagaacagcaatcccagctgtgtcctttcgagggtgagtgaaagcacatgctgtcctttacatgcttgaggcggacttgcctgtctcttcaggccggatgctcttcagggccctgtggggcttaaacacatgtactgagctagctccaatcttaatctgcacaacatcgcaacccctgagttcctattagttcttggtcccagtgtggatcgctctgagagaccacagctccctcctctggagtcccctctccgagctctccaagggaaaagacaaaggaagccgaactgccaagttgaagattttgcctcaggcaaaagttcttcgtgaccaggtgggtcttgtaatgcttggtgaggtggtcactcctcatgaagcgcttctgacactgggcgcactcgaagcgtttgtcccctgtgtgggtgcgagcatgccgttggagctcgtcactccgtgtgaacctcttcccacagaagaaccagttgcagacaaagggccgctcgccagtgtgcaggcgcacatgggcacgcagcaaggacgtcttacggaacgtcttgccacagtcggggatgtggcacacgtgcttcttcttgccctgctctccagacctcttctccccatccttgcagttgggacacgtgcaggccatgcggcgccgcttctccccgggctgggtctctccggccagggcttgttccatttgcagctggatctgggtggggctcagcccactgatggtcaggttgttcccagaaacattctgcactgtcagctgctgctgcccgcctgtgttggtgatggtgacaggcacgccctggacctggacaccattgatgttgatggtctgcattgcctgggcagctgccgccaactgggctgcattcaggctgatgatgctcccggctggggcaatctttggcaggggacgctcttttcggagaattgcagctgagtgctttttgctggtcccactcagatggggagcacgggatgcagggctgctacaggtggtgttagaggtggctgcagctgttgctggggggctgtcctggacaaggactgtctgcacctcaccggaaggcgtgcggatgtagacctgagtaggtgtcggctcagctgcctggatctgaaagttctgggagggcttctggggtacagtggggagggtggcagatgccgcctgcaccacccgcagagcctgctgggggatctgtaccacctgctgctgctcggccttggggggcaccacctggacctgctggaccacagctggctggcccccaccagggctctgaacaatgagcaggttatttcctgcctggatgatgttgtccgcggtggtctcgatcagcaccgtctccacctgctcagccacagccacagggggctgggaggcaggaaggctcttcttccttgctttcttgttagtcttagacagcggggttggggggctttcagtgaggagctgagtaggggccccggtgtcactggcgttcacaaggttgttgacgggcagagtgagcgtcacattgccgcccccacctgtcagcttcaccacattggccccgctctgcacgggggtggtggtcgtactcgacttctggatgggggctggcttgatggggacaggcttgtgactggacggtgagggggtgatgatggcttggttggtgccagggatgatctggatctggttggtgagattgggctgtacttggatggtttgggaattgcttgcctgaatctgagggaccgcctggtactggatattggcatttgatcgggtccctttgttgatcatggtgggattctggatagcgaacaccagctgccctccaggataggaggcgctcagttgtgacccctgaatctgaagtatatttcctttggaggacaagattccaaagctattcttgccggggctgagagggagaggggcaggtttgatagggacaagtttccgcggtgtgggctgtgggggagcaggaggtgtcacagcagcttcaactgctggagggccaattttgctacatgttgcagcaagcagggctaagggagatggctgggagtcctgggtggtggaggcggcaggctgcaggtagtcactgggactcacagcagcagtggcagccatgctggtctgtggatcgctcattacgacatcttcctccctggcctccgccgcctccgccgccaccgagagcctgacaccgcccgccaagcaaccgccaatcccggagcccgccaccgcccgagcgacggcagccttcaccaataagcgcttgg

SEQ ID NO: 15689 - RNA, 3635 nt, Homo sapiens
  source 1..3635: mol_type = other RNA
gctgggattacaggcatgagccactgtgcccggccagaaagatgattgtaaaaatggactgggtggtctgaaggaagggcaaggaagacccatttgctggttttgttaaagaaaaaaaaaaaagtacatataatgcctggatttgcctttgggagggaaatcctgcccagtccctctttcttccaggcatggaatcctaggctgtgggataatgagcacaatgccaagtgtcagctggacagagaggaagggcatgagggatgggctttggtgcacatgacgctggggacagtagaggacagaggaggaactacacatgtggggcccctacccttgagctgcacccagattttcatcaagggcccatcaggatcaggtgtctgtgggagcctcttgcctagggtgagcttagactgcatcacaccttcaacagttcccctgcaactctcaaataatggataggttaaagccagaggagggttaatttgcccacaagtctttctgtgctttccttgtgccatcactcagctaggcagaatacattctctcgctcttagccatcccaagggaggcagagatgatcagacataacttttgaacccccatctcactggagaagggaaatcctacatgggaaatgctcatcctgcccaacttggggctggcaccttcatttccaaatgatgctggggagtcaggtcagtttctgtactggaagcataaagcacatggcttgaaatcagctcccaggaaaggatcattctttgtgcctgagagcaaagccaagggaaacgtggcaaaaagaggtcactttgttaatattccccttctctccaccaatccccttattcagaatgcagcaaggcagttttctagtcatgcagtccacgcatgaggaataaatacacctcatgtcttccacctgctgccagtgcggtgatgagatgcagagctgaggggctgaggaagaggcttctgtgtcaaggtagattcagctggtggtctagtattgcccaaacgacttccgtagggataggaaaggcccctgcttgttaacaaagaagagggaaagggcagagaacctggatccatctgagatctgtgggctttttactttttcagccatttgagggttgactggctctaaggaaaagctgtttgctggcagacacaggtggctggtgacaaagggaacagagcaggggaatggatagctcaaaacgagcctcgccactcctgaacagaacagcaatcccagctgtgtcctttcgagggtgagtgaaagcacatgctgtcctttacatgcttgaggcggacttgcctgtctcttcaggccggatgctcttcagggccctgtggggcttaaacacatgtactgagctagctccaatcttaatctgcacaacatcgcaacccctgagttcctattagttcttggtcccagtgtggatcgctctgagagaccacagctccctcctctggagtcccctctccgagctctccaagggaaaagacaaaggaagccgaactgccaagttgaagattttgcctcaggcaaaagttcttcgtgaccaggtgggtcttgtaatgcttggtgaggtggtcactcctcatgaagcgcttctgacactgggcgcactcgaagcgtttgtcccctgtgtgggtgcgagcatgccgttggagctcgtcactccgtgtgaacctcttcccacagaagaaccagttgcagacaaagggccgctcgccagtgtgcaggcgcacatgggcacgcagcaaggacgtcttacggaacgtcttgccacagtcggggatgtggcacacgtgcttcttcttgccctgctctccagacctcttctccccatccttgcagttgggacacgtgcaggccatgcggcgccgcttctccccgggctgggtctctccggccagggcttgttccatttgcagctggatctgggtggggctcagcccactgatggtcaggttgttcccagaaacattctgcactgtcagctgctgctgcccgcctgtgttggtgatggtgacaggcacgccctggacctggacaccattgatgttgatggtctgcattgcctgggcagctgccgccaactgggctgcattcaggctgatgatgctcccggctggggcaatctttggcaggggacgctcttttcggagaattgcagctgagtgctttttgctggtcccactcagatggggagcacgggatgcagggctgctacaggtggtgttagaggtggctgcagctgttgctggggggctgtcctggacaaggactgtctgcacctcaccggaaggcgtgcggatgtagacctgagtaggtgtcggctcagctgcctggatctgaaagttctgggagggcttctggggtacagtggggagggtggcagatgccgcctgcaccacccgcagagcctgctgggggatctgtaccacctgctgctgctcggccttggggggcaccacctggacctgctggaccacagctggctggcccccaccagggctctgaacaatgagcaggttatttcctgcctggatgatgttgtccgcggtggtctcgatcagcaccgtctccacctgctcagccacagccacagggggctgggaggcaggaaggctcttcttccttgctttcttgttagtcttagacagcggggttggggggctttcagtgaggagctgagtaggggccccggtgtcactggcgttcacaaggttgttgacgggcagagtgagcgtcacattgccgcccccacctgtcagcttcaccacattggccccgctctgcacgggggtggtggtcgtactcgacttctggatgggggctggcttgatggggacaggcttgtgactggacggtgagggggtgatgatggcttggttggtgccagggatgatctggatctggttggtgagattgggctgtacttggatggtttgggaattgcttgcctgaatctgagggaccgcctggtactggatattggcatttgatcgggtccctttgttgatcatggtgggattctggatagcgaacaccagctgccctccaggataggaggcgctcagttgtgacccctgaatctgaagtatatttcctttggaggacaagattccaaagctattcttgccggggctgagagggagaggggcaggtttgatagggacaagtttccgcggtgtgggctgtgggggagcaggaggtgtcacagcagcttcaactgctggagggccaattttgctacatgttgcagcaagcagggctaagggagatggctgggagtcctgggtggtggaggcggcaggctgcaggtagtcactgggactcacagcagcagtggcagccatgctggtctgtggatctaaatgagattctgactgtgtggttcattagtgggatggtccctcttagcctcctcctagtgccctcaatcgtcccagccaatgataatccatttccaacaggtattaacgcctgttagaagccactggaacactgacatcatcagcccaattgataggttgtctgatagattcgcccccgctcattacgacatcttcctccctggcctccgccgcctccgccgccaccgagagcctgacaccgc

SEQ ID NO: 15690 - RNA, 3524 nt, Homo sapiens
  source 1..3524: mol_type = other RNA
gctgggattacaggcatgagccactgtgcccggccagaaagatgattgtaaaaatggactgggtggtctgaaggaagggcaaggaagacccatttgctggttttgttaaagaaaaaaaaaaaagtacatataatgcctggatttgcctttgggagggaaatcctgcccagtccctctttcttccaggcatggaatcctaggctgtgggataatgagcacaatgccaagtgtcagctggacagagaggaagggcatgagggatgggctttggtgcacatgacgctggggacagtagaggacagaggaggaactacacatgtggggcccctacccttgagctgcacccagattttcatcaagggcccatcaggatcaggtgtctgtgggagcctcttgcctagggtgagcttagactgcatcacaccttcaacagttcccctgcaactctcaaataatggataggttaaagccagaggagggttaatttgcccacaagtctttctgtgctttccttgtgccatcactcagctaggcagaatacattctctcgctcttagccatcccaagggaggcagagatgatcagacataacttttgaacccccatctcactggagaagggaaatcctacatgggaaatgctcatcctgcccaacttggggctggcaccttcatttccaaatgatgctggggagtcaggtcagtttctgtactggaagcataaagcacatggcttgaaatcagctcccaggaaaggatcattctttgtgcctgagagcaaagccaagggaaacgtggcaaaaagaggtcactttgttaatattccccttctctccaccaatccccttattcagaatgcagcaaggcagttttctagtcatgcagtccacgcatgaggaataaatacacctcatgtcttccacctgctgccagtgcggtgatgagatgcagagctgaggggctgaggaagaggcttctgtgtcaaggtagattcagctggtggtctagtattgcccaaacgacttccgtagggataggaaaggcccctgcttgttaacaaagaagagggaaagggcagagaacctggatccatctgagatctgtgggctttttactttttcagccatttgagggttgactggctctaaggaaaagctgtttgctggcagacacaggtggctggtgacaaagggaacagagcaggggaatggatagctcaaaacgagcctcgccactcctgaacagaacagcaatcccagctgtgtcctttcgagggtgagtgaaagcacatgctgtcctttacatgcttgaggcggacttgcctgtctcttcaggccggatgctcttcagggccctgtggggcttaaacacatgtactgagctagctccaatcttaatctgcacaacatcgcaacccctgagttcctattagttcttggtcccagtgtggatcgctctgagagaccacagctccctcctctggagtcccctctccgagctctccaagggaaaagacaaaggaagccgaactgccaagttgaagattttgcctcaggcaaaagttcttcgtgaccaggtgggtcttgtaatgcttggtgaggtggtcactcctcatgaagcgcttctgacactgggcgcactcgaagcgtttgtcccctgtgtgggtgcgagcatgccgttggagctcgtcactccgtgtgaacctcttcccacagaagaaccagttgcagacaaagggccgctcgccagtgtgcaggcgcacatgggcacgcagcaaggacgtcttacggaacgtcttgccacagtcggggatgtggcacacgtgcttcttcttgccctgctctccagacctcttctccccatccttgcagttgggacacgtgcaggccatgcggcgccgcttctccccgggctgggtctctccggccagggcttgttccatttgcagctggatctgggtggggctcagcccactgatggtcaggttgttcccagaaacattctgcactgtcagctgctgctgcccgcctgtgttggtgatggtgacaggcacgccctggacctggacaccattgatgttgatggtctgcattgcctgggcagctgccgccaactgggctgcattcaggctgatgatgctcccggctggggcaatctttggcaggggacgctcttttcggagaattgcagctgagtgctttttgctggtcccactcagatggggagcacgggatgcagggctgctacaggtggtgttagaggtggctgcagctgttgctggggggctgtcctggacaaggactgtctgcacctcaccggaaggcgtgcggatgtagacctgagtaggtgtcggctcagctgcctggatctgaaagttctgggagggcttctggggtacagtggggagggtggcagatgccgcctgcaccacccgcagagcctgctgggggatctgtaccacctgctgctgctcggccttggggggcaccacctggacctgctggaccacagctggctggcccccaccagggctctgaacaatgagcaggttatttcctgcctggatgatgttgtccgcggtggtctcgatcagcaccgtctccacctgctcagccacagccacagggggctgggaggcaggaaggctcttcttccttgctttcttgttagtcttagacagcggggttggggggctttcagtgaggagctgagtaggggccccggtgtcactggcgttcacaaggttgttgacgggcagagtgagcgtcacattgccgcccccacctgtcagcttcaccacattggccccgctctgcacgggggtggtggtcgtactcgacttctggatgggggctggcttgatggggacaggcttgtgactggacggtgagggggtgatgatggcttggttggtgccagggatgatctggatctggttggtgagattgggctgtacttggatggtttgggaattgcttgcctgaatctgagggaccgcctggtactggatattggcatttgatcgggtccctttgttgatcatggtgggattctggatagcgaacaccagctgccctccaggataggaggcgctcagttgtgacccctgaatctgaagtatatttcctttggaggacaagattccaaagctattcttgccggggctgagagggagaggggcaggtttgatagggacaagtttccgcggtgtgggctgtgggggagcaggaggtgtcacagcagcttcaactgctggagggccaattttgctacatgttgcagcaagcagggctaagggagatggctgggagtcctgggtggtggaggcggcaggctgcaggtagtcactgggactcacagcagcagtggcagccatgctggtctgtggatctaaatgagattctgactgtgtggttcattagtgggatggtccctcttagcctcctcctagtgccctcgctcattacgacatcttcctccctggcctccgccgcctccgccgccaccgagagcctgacaccgccc

SEQ ID NO: 15691 - RNA, 5231 nt, Homo sapiens
  source 1..5231: mol_type = other RNA
gctgggattacaggcatgagccactgtgcccggccagaaagatgattgtaaaaatggactgggtggtctgaaggaagggcaaggaagacccatttgctggttttgttaaagaaaaaaaaaaaagtacatataatgcctggatttgcctttgggagggaaatcctgcccagtccctctttcttccaggcatggaatcctaggctgtgggataatgagcacaatgccaagtgtcagctggacagagaggaagggcatgagggatgggctttggtgcacatgacgctggggacagtagaggacagaggaggaactacacatgtggggcccctacccttgagctgcacccagattttcatcaagggcccatcaggatcaggtgtctgtgggagcctcttgcctagggtgagcttagactgcatcacaccttcaacagttcccctgcaactctcaaataatggataggttaaagccagaggagggttaatttgcccacaagtctttctgtgctttccttgtgccatcactcagctaggcagaatacattctctcgctcttagccatcccaagggaggcagagatgatcagacataacttttgaacccccatctcactggagaagggaaatcctacatgggaaatgctcatcctgcccaacttggggctggcaccttcatttccaaatgatgctggggagtcaggtcagtttctgtactggaagcataaagcacatggcttgaaatcagctcccaggaaaggatcattctttgtgcctgagagcaaagccaagggaaacgtggcaaaaagaggtcactttgttaatattccccttctctccaccaatccccttattcagaatgcagcaaggcagttttctagtcatgcagtccacgcatgaggaataaatacacctcatgtcttccacctgctgccagtgcggtgatgagatgcagagctgaggggctgaggaagaggcttctgtgtcaaggtagattcagctggtggtctagtattgcccaaacgacttccgtagggataggaaaggcccctgcttgttaacaaagaagagggaaagggcagagaacctggatccatctgagatctgtgggctttttactttttcagccatttgagggttgactggctctaaggaaaagctgtttgctggcagacacaggtggctggtgacaaagggaacagagcaggggaatggatagctcaaaacgagcctcgccactcctgaacagaacagcaatcccagctgtgtcctttcgagggtgagtgaaagcacatgctgtcctttacatgcttgaggcggacttgcctgtctcttcaggccggatgctcttcagggccctgtggggcttaaacacatgtactgagctagctccaatcttaatctgcacaacatcgcaacccctgagttcctattagttcttggtcccagtgtggatcgctctgagagaccacagctccctcctctggagtcccctctccgagctctccaagggaaaagacaaaggaagccgaactgccaagttgaagattttgcctcaggcaaaagttcttcgtgaccaggtgggtcttgtaatgcttggtgaggtggtcactcctcatgaagcgcttctgacactgggcgcactcgaagcgtttgtcccctgtgtgggtgcgagcatgccgttggagctcgtcactccgtgtgaacctcttcccacagaagaaccagttgcagacaaagggccgctcgccagtgtgcaggcgcacatgggcacgcagcaaggacgtcttacggaacgtcttgccacagtcggggatgtggcacacgtgcttcttcttgccctgctctccagacctcttctccccatccttgcagttgggacacgtgcaggccatgcggcgccgcttctccccgggctgggtctctccggccagggcttgttccatttgcagctggatctgggtggggctcagcccactgatggtcaggttgttcccagaaacattctgcactgtcagctgctgctgcccgcctgtgttggtgatggtgacaggcacgccctggacctggacaccattgatgttgatggtctgcattgcctgggcagctgccgccaactgggctgcattcaggctgatgatgctcccggctggggcaatctttggcaggggacgctcttttcggagaattgcagctgagtgctttttgctggtcccactcagatggggagcacgggatgcagggctgctacaggtggtgttagaggtggctgcagctgttgctggggggctgtcctggacaaggactgtctgcacctcaccggaaggcgtgcggatgtagacctgagtaggtgtcggctcagctgcctggatctgaaagttctgggagggcttctggggtacagtggggagggtggcagatgccgcctgcaccacccgcagagcctgctgggggatctgtaccacctgctgctgctcggccttggggggcaccacctggacctgctggaccacagctggctggcccccaccagggctctgaacaatgagcaggttatttcctgcctggatgatgttgtccgcggtggtctcgatcagcaccgtctccacctgctcagccacagccacagggggctgggaggcaggaaggctcttcttccttgctttcttgttagtcttagacagcggggttggggggctttcagtgaggagctgagtaggggccccggtgtcactggcgttcacaaggttgttgacgggcagagtgagcgtcacattgccgcccccacctgtcagcttcaccacattggccccgctctgcacgggggtggtggtcgtactcgacttctggatgggggctggcttgatggggacaggcttgtgactggacggtgagggggtgatgatggcttggttggtgccagggatgatctggatctggttggtgagattgggctgtacttggatggtttgggaattgcttgcctgaatctgagggaccgcctggtactggatattggcatttgatcgggtccctttgttgatcatggtgggattctggatagcgaacaccagctgccctccaggataggaggcgctcagttgtgacccctgaatctgaagtatatttcctttggaggacaagattccaaagctattcttgccggggctgagagggagaggggcaggtttgatagggacaagtttccgcggtgtgggctgtgggggagcaggaggtgtcacagcagcttcaactgctggagggccaattttgctacatgttgcagcaagcagggctaagggagatggctgggagtcctgggtggtggaggcggcaggctgcaggtagtcactgggactcacagcagcagtggcagccatgctggtctgtggatcttccacaggctgccaactcataggcctgtgtctggcccagatctctgctccacgtgttagacctgtacatccagccctctgtgggtcttccattagggctggccacagacacctggggcactgagcgacagctttgcccattctttgtccagccttctcaccctcagccaccacaggccttcttccagatccttgaaaaacttcagtgtctgcagctgtctttccttgcttacagctctttctgttctcttcactagctaagacctcacccttcaggtctctggctgtttgactttcccagcataatttaagagccattatgtaacaggcatgccatttcctcagagaggcctttctggacccctgagatgaggctaactcctttgggaacactcaccactcattaactaatcatgagcccaatgtatgcgagggctccccagggtgggccatgtctgtttacaccactgaactgcagacaccaaggcctggcacatggctcacggacaccttcagtgcctatgggctgtatgaatatcctgggttaaagcagcctctcttctggtatctccaatcaggacaaaacctgagtatccccctcactgccaaccaatcatcaagtcctcatgattccacctcatagacaaatctccctatagtgtacccaggctccccatcctcatcaccatgatccacctgagatactgcctacggcctctaaaactgcttcctggcctctggcctcccccttagtcagcctccacaatttggttagaaggctctttttaaagtgcaaatcccatccagctactctcctaattaaccccctcaattgttccctgatgctcttgtgataaacttataaaggccagaacaacctgtccctccctggtcctccctcctgacctctttcccttccaactctcccaacacacacttcagtttttcatttctggaattaaaacacgccaccctgtctcacttggagcctgaagcacactctctcccatttgcccggccagctcctgtcctttagagctcatttatactctcactcagcgaaagcctttcctgacctcctcccacctcaaatctggggcaggtgaccctgctacctgccagtgcatactccaggcacccttcggcactgtcccatcaacacagagctgggagtgtgtccctgtcccacggtctttctaggcctgacttggggagagcacgtaacaggaagagagacctctgagccctggccaccaggctgcaggctgttcgactgttcctttcactgagaatgctactcttgagacccagcaaatgagaaaacgcgcctacagaaataccacaacagtaggctttaggaagctttttcttctggagagaactaggctccatctccacaacccaggccttgggggtaactcggctttttttgcctgtgggttcctgccatcgtgggtctggctttcttggctttttgctatggtatttcccctggaggaatttcacactgtgcaaacagtctttctcttggctattttggtcagctcagctgggccgtaagccaacaaagcagtttctaagcccaggcttttccagttgcctagcctggaagaattcagagctggtgagggaaaagcatgccctggctggttttagagaacaaagttggacctcaaagaaagctcacaaatggggtatgagaatccatttggatgaagaaagcagcaaccttggtagtgaaagactccaaattgtgctgaatatttcaatgagaggcaaacctcagcaatcataataactattataaggtgggcacggtggctcatgcctgtaataccagc

SEQ ID NO: 15692 - RNA, 5159 nt, Homo sapiens
  source 1..5159: mol_type = other RNA
gctgggattacaggcatgagccactgtgcccggccagaaagatgattgtaaaaatggactgggtggtctgaaggaagggcaaggaagacccatttgctggttttgttaaagaaaaaaaaaaaagtacatataatgcctggatttgcctttgggagggaaatcctgcccagtccctctttcttccaggcatggaatcctaggctgtgggataatgagcacaatgccaagtgtcagctggacagagaggaagggcatgagggatgggctttggtgcacatgacgctggggacagtagaggacagaggaggaactacacatgtggggcccctacccttgagctgcacccagattttcatcaagggcccatcaggatcaggtgtctgtgggagcctcttgcctagggtgagcttagactgcatcacaccttcaacagttcccctgcaactctcaaataatggataggttaaagccagaggagggttaatttgcccacaagtctttctgtgctttccttgtgccatcactcagctaggcagaatacattctctcgctcttagccatcccaagggaggcagagatgatcagacataacttttgaacccccatctcactggagaagggaaatcctacatgggaaatgctcatcctgcccaacttggggctggcaccttcatttccaaatgatgctggggagtcaggtcagtttctgtactggaagcataaagcacatggcttgaaatcagctcccaggaaaggatcattctttgtgcctgagagcaaagccaagggaaacgtggcaaaaagaggtcactttgttaatattccccttctctccaccaatccccttattcagaatgcagcaaggcagttttctagtcatgcagtccacgcatgaggaataaatacacctcatgtcttccacctgctgccagtgcggtgatgagatgcagagctgaggggctgaggaagaggcttctgtgtcaaggtagattcagctggtggtctagtattgcccaaacgacttccgtagggataggaaaggcccctgcttgttaacaaagaagagggaaagggcagagaacctggatccatctgagatctgtgggctttttactttttcagccatttgagggttgactggctctaaggaaaagctgtttgctggcagacacaggtggctggtgacaaagggaacagagcaggggaatggatagctcaaaacgagcctcgccactcctgaacagaacagcaatcccagctgtgtcctttcgagggtgagtgaaagcacatgctgtcctttacatgcttgaggcggacttgcctgtctcttcaggccggatgctcttcagggccctgtggggcttggtcccagtgtggatcgctctgagagaccacagctccctcctctggagtcccctctccgagctctccaagggaaaagacaaaggaagccgaactgccaagttgaagattttgcctcaggcaaaagttcttcgtgaccaggtgggtcttgtaatgcttggtgaggtggtcactcctcatgaagcgcttctgacactgggcgcactcgaagcgtttgtcccctgtgtgggtgcgagcatgccgttggagctcgtcactccgtgtgaacctcttcccacagaagaaccagttgcagacaaagggccgctcgccagtgtgcaggcgcacatgggcacgcagcaaggacgtcttacggaacgtcttgccacagtcggggatgtggcacacgtgcttcttcttgccctgctctccagacctcttctccccatccttgcagttgggacacgtgcaggccatgcggcgccgcttctccccgggctgggtctctccggccagggcttgttccatttgcagctggatctgggtggggctcagcccactgatggtcaggttgttcccagaaacattctgcactgtcagctgctgctgcccgcctgtgttggtgatggtgacaggcacgccctggacctggacaccattgatgttgatggtctgcattgcctgggcagctgccgccaactgggctgcattcaggctgatgatgctcccggctggggcaatctttggcaggggacgctcttttcggagaattgcagctgagtgctttttgctggtcccactcagatggggagcacgggatgcagggctgctacaggtggtgttagaggtggctgcagctgttgctggggggctgtcctggacaaggactgtctgcacctcaccggaaggcgtgcggatgtagacctgagtaggtgtcggctcagctgcctggatctgaaagttctgggagggcttctggggtacagtggggagggtggcagatgccgcctgcaccacccgcagagcctgctgggggatctgtaccacctgctgctgctcggccttggggggcaccacctggacctgctggaccacagctggctggcccccaccagggctctgaacaatgagcaggttatttcctgcctggatgatgttgtccgcggtggtctcgatcagcaccgtctccacctgctcagccacagccacagggggctgggaggcaggaaggctcttcttccttgctttcttgttagtcttagacagcggggttggggggctttcagtgaggagctgagtaggggccccggtgtcactggcgttcacaaggttgttgacgggcagagtgagcgtcacattgccgcccccacctgtcagcttcaccacattggccccgctctgcacgggggtggtggtcgtactcgacttctggatgggggctggcttgatggggacaggcttgtgactggacggtgagggggtgatgatggcttggttggtgccagggatgatctggatctggttggtgagattgggctgtacttggatggtttgggaattgcttgcctgaatctgagggaccgcctggtactggatattggcatttgatcgggtccctttgttgatcatggtgggattctggatagcgaacaccagctgccctccaggataggaggcgctcagttgtgacccctgaatctgaagtatatttcctttggaggacaagattccaaagctattcttgccggggctgagagggagaggggcaggtttgatagggacaagtttccgcggtgtgggctgtgggggagcaggaggtgtcacagcagcttcaactgctggagggccaattttgctacatgttgcagcaagcagggctaagggagatggctgggagtcctgggtggtggaggcggcaggctgcaggtagtcactgggactcacagcagcagtggcagccatgctggtctgtggatcttccacaggctgccaactcataggcctgtgtctggcccagatctctgctccacgtgttagacctgtacatccagccctctgtgggtcttccattagggctggccacagacacctggggcactgagcgacagctttgcccattctttgtccagccttctcaccctcagccaccacaggccttcttccagatccttgaaaaacttcagtgtctgcagctgtctttccttgcttacagctctttctgttctcttcactagctaagacctcacccttcaggtctctggctgtttgactttcccagcataatttaagagccattatgtaacaggcatgccatttcctcagagaggcctttctggacccctgagatgaggctaactcctttgggaacactcaccactcattaactaatcatgagcccaatgtatgcgagggctccccagggtgggccatgtctgtttacaccactgaactgcagacaccaaggcctggcacatggctcacggacaccttcagtgcctatgggctgtatgaatatcctgggttaaagcagcctctcttctggtatctccaatcaggacaaaacctgagtatccccctcactgccaaccaatcatcaagtcctcatgattccacctcatagacaaatctccctatagtgtacccaggctccccatcctcatcaccatgatccacctgagatactgcctacggcctctaaaactgcttcctggcctctggcctcccccttagtcagcctccacaatttggttagaaggctctttttaaagtgcaaatcccatccagctactctcctaattaaccccctcaattgttccctgatgctcttgtgataaacttataaaggccagaacaacctgtccctccctggtcctccctcctgacctctttcccttccaactctcccaacacacacttcagtttttcatttctggaattaaaacacgccaccctgtctcacttggagcctgaagcacactctctcccatttgcccggccagctcctgtcctttagagctcatttatactctcactcagcgaaagcctttcctgacctcctcccacctcaaatctggggcaggtgaccctgctacctgccagtgcatactccaggcacccttcggcactgtcccatcaacacagagctgggagtgtgtccctgtcccacggtctttctaggcctgacttggggagagcacgtaacaggaagagagacctctgagccctggccaccaggctgcaggctgttcgactgttcctttcactgagaatgctactcttgagacccagcaaatgagaaaacgcgcctacagaaataccacaacagtaggctttaggaagctttttcttctggagagaactaggctccatctccacaacccaggccttgggggtaactcggctttttttgcctgtgggttcctgccatcgtgggtctggctttcttggctttttgctatggtatttcccctggaggaatttcacactgtgcaaacagtctttctcttggctattttggtcagctcagctgggccgtaagccaacaaagcagtttctaagcccaggcttttccagttgcctagcctggaagaattcagagctggtgagggaaaagcatgccctggctggttttagagaacaaagttggacctcaaagaaagctcacaaatggggtatgagaatccatttggatgaagaaagcagcaaccttggtagtgaaagactccaaattgtgctgaatatttcaatgagaggcaaacctcagcaatcataataactattataaggtgggcacggtggctcatgcctgtaataccagc

SEQ ID NO: 15693 - RNA, 5151 nt, Homo sapiens
  source 1..5151: mol_type = other RNA
gctgggattacaggcatgagccactgtgcccggccagaaagatgattgtaaaaatggactgggtggtctgaaggaagggcaaggaagacccatttgctggttttgttaaagaaaaaaaaaaaagtacatataatgcctggatttgcctttgggagggaaatcctgcccagtccctctttcttccaggcatggaatcctaggctgtgggataatgagcacaatgccaagtgtcagctggacagagaggaagggcatgagggatgggctttggtgcacatgacgctggggacagtagaggacagaggaggaactacacatgtggggcccctacccttgagctgcacccagattttcatcaagggcccatcaggatcaggtgtctgtgggagcctcttgcctagggtgagcttagactgcatcacaccttcaacagttcccctgcaactctcaaataatggataggttaaagccagaggagggttaatttgcccacaagtctttctgtgctttccttgtgccatcactcagctaggcagaatacattctctcgctcttagccatcccaagggaggcagagatgatcagacataacttttgaacccccatctcactggagaagggaaatcctacatgggaaatgctcatcctgcccaacttggggctggcaccttcatttccaaatgatgctggggagtcaggtcagtttctgtactggaagcataaagcacatggcttgaaatcagctcccaggaaaggatcattctttgtgcctgagagcaaagccaagggaaacgtggcaaaaagaggtcactttgttaatattccccttctctccaccaatccccttattcagaatgcagcaaggcagttttctagtcatgcagtccacgcatgaggaataaatacacctcatgtcttccacctgctgccagtgcggtgatgagatgcagagctgaggggctgaggaagaggcttctgtgtcaaggtagattcagctggtggtctagtattgcccaaacgacttccgtagggataggaaaggcccctgcttgttaacaaagaagagggaaagggcagagaacctggatccatctgagatctgtgggctttttactttttcagccatttgagggttgactggctctaaggaaaagctgtttgctggcagacacaggtggctggtgacaaagggaacagagcaggggaatggatagctcaaaacgagcctcgccactcctgaacagaacagcaatcccagctgtgtcctttcgagggtgagtgaaagcacatgctgtcctttacatgcttgaggcggacttgcctgtctcttcaggccggatgctcttcagggcccttggtcccagtgtggatcgctctgagagaccacagctccctcctctggagtcccctctccgagctctccaagggaaaagacaaaggaagccgaactgccaagttgaagattttgcctcaggcaaaagttcttcgtgaccaggtgggtcttgtaatgcttggtgaggtggtcactcctcatgaagcgcttctgacactgggcgcactcgaagcgtttgtcccctgtgtgggtgcgagcatgccgttggagctcgtcactccgtgtgaacctcttcccacagaagaaccagttgcagacaaagggccgctcgccagtgtgcaggcgcacatgggcacgcagcaaggacgtcttacggaacgtcttgccacagtcggggatgtggcacacgtgcttcttcttgccctgctctccagacctcttctccccatccttgcagttgggacacgtgcaggccatgcggcgccgcttctccccgggctgggtctctccggccagggcttgttccatttgcagctggatctgggtggggctcagcccactgatggtcaggttgttcccagaaacattctgcactgtcagctgctgctgcccgcctgtgttggtgatggtgacaggcacgccctggacctggacaccattgatgttgatggtctgcattgcctgggcagctgccgccaactgggctgcattcaggctgatgatgctcccggctggggcaatctttggcaggggacgctcttttcggagaattgcagctgagtgctttttgctggtcccactcagatggggagcacgggatgcagggctgctacaggtggtgttagaggtggctgcagctgttgctggggggctgtcctggacaaggactgtctgcacctcaccggaaggcgtgcggatgtagacctgagtaggtgtcggctcagctgcctggatctgaaagttctgggagggcttctggggtacagtggggagggtggcagatgccgcctgcaccacccgcagagcctgctgggggatctgtaccacctgctgctgctcggccttggggggcaccacctggacctgctggaccacagctggctggcccccaccagggctctgaacaatgagcaggttatttcctgcctggatgatgttgtccgcggtggtctcgatcagcaccgtctccacctgctcagccacagccacagggggctgggaggcaggaaggctcttcttccttgctttcttgttagtcttagacagcggggttggggggctttcagtgaggagctgagtaggggccccggtgtcactggcgttcacaaggttgttgacgggcagagtgagcgtcacattgccgcccccacctgtcagcttcaccacattggccccgctctgcacgggggtggtggtcgtactcgacttctggatgggggctggcttgatggggacaggcttgtgactggacggtgagggggtgatgatggcttggttggtgccagggatgatctggatctggttggtgagattgggctgtacttggatggtttgggaattgcttgcctgaatctgagggaccgcctggtactggatattggcatttgatcgggtccctttgttgatcatggtgggattctggatagcgaacaccagctgccctccaggataggaggcgctcagttgtgacccctgaatctgaagtatatttcctttggaggacaagattccaaagctattcttgccggggctgagagggagaggggcaggtttgatagggacaagtttccgcggtgtgggctgtgggggagcaggaggtgtcacagcagcttcaactgctggagggccaattttgctacatgttgcagcaagcagggctaagggagatggctgggagtcctgggtggtggaggcggcaggctgcaggtagtcactgggactcacagcagcagtggcagccatgctggtctgtggatcttccacaggctgccaactcataggcctgtgtctggcccagatctctgctccacgtgttagacctgtacatccagccctctgtgggtcttccattagggctggccacagacacctggggcactgagcgacagctttgcccattctttgtccagccttctcaccctcagccaccacaggccttcttccagatccttgaaaaacttcagtgtctgcagctgtctttccttgcttacagctctttctgttctcttcactagctaagacctcacccttcaggtctctggctgtttgactttcccagcataatttaagagccattatgtaacaggcatgccatttcctcagagaggcctttctggacccctgagatgaggctaactcctttgggaacactcaccactcattaactaatcatgagcccaatgtatgcgagggctccccagggtgggccatgtctgtttacaccactgaactgcagacaccaaggcctggcacatggctcacggacaccttcagtgcctatgggctgtatgaatatcctgggttaaagcagcctctcttctggtatctccaatcaggacaaaacctgagtatccccctcactgccaaccaatcatcaagtcctcatgattccacctcatagacaaatctccctatagtgtacccaggctccccatcctcatcaccatgatccacctgagatactgcctacggcctctaaaactgcttcctggcctctggcctcccccttagtcagcctccacaatttggttagaaggctctttttaaagtgcaaatcccatccagctactctcctaattaaccccctcaattgttccctgatgctcttgtgataaacttataaaggccagaacaacctgtccctccctggtcctccctcctgacctctttcccttccaactctcccaacacacacttcagtttttcatttctggaattaaaacacgccaccctgtctcacttggagcctgaagcacactctctcccatttgcccggccagctcctgtcctttagagctcatttatactctcactcagcgaaagcctttcctgacctcctcccacctcaaatctggggcaggtgaccctgctacctgccagtgcatactccaggcacccttcggcactgtcccatcaacacagagctgggagtgtgtccctgtcccacggtctttctaggcctgacttggggagagcacgtaacaggaagagagacctctgagccctggccaccaggctgcaggctgttcgactgttcctttcactgagaatgctactcttgagacccagcaaatgagaaaacgcgcctacagaaataccacaacagtaggctttaggaagctttttcttctggagagaactaggctccatctccacaacccaggccttgggggtaactcggctttttttgcctgtgggttcctgccatcgtgggtctggctttcttggctttttgctatggtatttcccctggaggaatttcacactgtgcaaacagtctttctcttggctattttggtcagctcagctgggccgtaagccaacaaagcagtttctaagcccaggcttttccagttgcctagcctggaagaattcagagctggtgagggaaaagcatgccctggctggttttagagaacaaagttggacctcaaagaaagctcacaaatggggtatgagaatccatttggatgaagaaagcagcaaccttggtagtgaaagactccaaattgtgctgaatatttcaatgagaggcaaacctcagcaatcataataactattataaggtgggcacggtggctcatgcctgtaataccagc

SEQ ID NO: 15694 - RNA, 2845 nt, Homo sapiens
  source 1..2845: mol_type = other RNA
gctgggattacaggcatgagccactgtgcccggcccaactctcattgttctctaccacacgactttcctcaagcatttgcttaccctgaaatacagtccctgaaaggcagagtacatggttgattatgtcctttttttgtgtgtgggcggggctaagtctattttcagagtaatgagtagccctagcagccatgaaaagtatcaacgagttgtttttgttttgaggggtgttacgaccttatggtttttaaagatattttgatgtgtttcaatccactgcagtcatcatccgtttgcagcctctctttggtagcccatgcccctggagggtccttgttttcaggcaagaagatatctcagctcatcatgtacatttctgccccagccctagaatcagacatttctccaaggagtcctggttcctttcagtgggaaatgttcttagagacattataatctggacactaacgatgtctgtggaatttttacaagatcgccttggcttctctgtgcatgatgaactggagggacaagaccaggccagagagacaggtcaagagactttcgcagtggcccaagtgagatataacagtggcttgaacttgatcttaggtaaatcacttagcgcaatgcttggtacatgatggagagcaccataaatggtagcacactctttcatcaatgacttgatctgtattagtttacttaaactccaaaactgtatgaggaagacttccttatcattgtatacatgagaaaacccaagctcagagaggtgaggaaacttgttcaaggtcacacaggaaatgaacagcagaaatagaacctgaatccagatctcgtgctctaaccaatgcactgtgtcgcccagagggttcttggtttcacactcaaaaatgacttacattttggtgcaaaacctgatccatcacgagttcatggcgattctcctggttgtgccctcaggtttgtgattttatttgcttcccagtgagatcataaacccacgagggcagggctgggccattcctgcctgtttgctccatgtctccagcagcgtgtaccacacctggcaggtgctcaggaaatacctgctgatgaatgagtgaatggctgaagaaggcaaattcacagcacagcagggggagaagcgaagaaggataggattccacctgtgaagatggcaaggaccagaacttaggagagctgaacagtggacttcagcaatttctgcagggataattcaagtgagaggctagccagacagatcagactgataggcctttagactgcggaacatgttttccattggaggtggaaaaacggctcctcttaccttccttcaaggcaggggccgatctggaaccattcaggccagttttgcttgggatggcagattcaccacatcaagaatttgatctgaaccaggcatggtggcttatgcctgtaatcccagaactttgggaggaagaggtgggaagattgcttgaggacaggagttcaagaccagcctgggcaacacagaaagaccctatctctacaaaatataaaaaagattagctagatgtcgtggtgtgcacctgtagtcccagctatttgggaggctaaaacaggaggattgcttgatcccaggagttcgaggctgctgtcagttacaattgtgccactggactccagcctgggtgacagagagagaccttgtctctacacacacaaaaaaaataaaaaataaaaagaaagaaaaaagaagtttggtttgtctcaacaggcattaattgagcacctacagtgtaccaggcattgtggatgtgcatctttctgggtctatactctcagagggccctgggagactcaatcatttgagtaatttcctggctgagggagaagctgaaatgtacaggcttctcttaaatatgttttgctccctgaagttgttccaaaatcagaggccttgaatgctgtacacccgtactctaggatggaatggtttgggatttggcacaaaaccagagatgtagtaatcttttgcttactctagcagtactggctgggattccctgaagacccagatgctctgacatgttgtaagtttgaaaactgctgaccctcttttgggtgtctttttcaggctctgattccaccaatccaatagggtagcccattaaacaattgaatcaacgacctggtcacctccgcctatgacaaatctagctttagagtcaggtagcccagggtcgaatgccatgtatacctccaagctgtgtgacttcaaacaagtcactccacctctctggacattggattctcatgtgtgaaatgggatacttgtaaacaagatgcttatagtggaaggcattattggtattattaattattaggacaaagctcttactcaggagttcaagatcagcctgggcaacaaagtgagatcctgtctctacagaaaaaaaaaaaacccaaaaaaccaaaaattagctgggcatggtggcacacgcctgtagtcccagctactctggaggctgaggtaggaggatggcttcagcctgggaggcagaggttgcagtgagccaagatcatgccactgcactctggcctgggtgatagatccagaattcgccaggactgagcagtttctcgtgttcattgtggtgaaggccacgatcactctttcaacaggcagctgttgcttgggttaggtttgcaagacataaaaatagctttgtctggcatctggttttcgggtccgctgggttatttcagcgaagggcagcagcttgtcatgatagcgtccacagaggttcactggaagggctcgtctggccttccctgctcatggaatcaaact

SEQ ID NO: 15695 - RNA, 2450 nt, Homo sapiens
  source 1..2450: mol_type = other RNA
gctgggattacaggcatgagccactgtgcccggccgctttctaagctttgtgaagagtgggttgactattcagatctctgcttctgtcccgctgtgccaagtgctggggcagacacaggcagagagtggacagcggcacggtgcctgctgctagccatttctatgcaaaaccagctttctggtcccatcctggaggccaattctaggcacctgggtgggcctgggaacctgtgaaccaagtaaactgacttggacacccccctaccccgccaggcctgtcctagcagccccacacaataccctcatgtcctgtccccaaacaccgccatcctcaaacacatgtgctctgtttccaggccgggccgggatcagatgggaagtggaacctcgtcatgagcagaaactgtttccctacgaagagcacttggagatggcaatgctgaatctcaccctgtaggactcacacacgactccaacgggattgtgagaatcaagtcactctcatgggaagaatttttatatgggaaagcggataaaactttcattggactggaatgtttggagaatgttaatttccaaatcaggaaccacaaactgccctctaataagacatcggctatctaagcgtgtgggtgccccctttctgccagcagttctggttcttaagaaaatcaccataaatcagacatgaaaattctggctccaaaaatagcattttctttgtgcaaataaaaacgtgtgtatcaagtatgatgttcccccaacgtggacacactcagttcctcacaaagccaagcccactgcagctgccacatccctgggcttacggtgcagcaggtgcttttttcaagacaggaatcaaaatgttaggaacacggcagaaaggggacacctggagaccaaacgcaggatgaggagttctgcagaggtcacagggaagtcacagaacagtaatacgctagcaggggcatggggcgtgaagaacagaagaagagaggaagcgtttccaagcctccagagaagaaatcaaggccaaccaaagcttcccgggtcacagaaccaattcttttaccaggcagtaccactgctgtcatttcagcttctggccactgggaggtgctgctcgaaagggtttgccctgagactccaagaagaagctgcgggaaggacagcaggggtcctggggttttagcctctggcccaggagttatgtgtccataaccaaagggagcacagtctgcacccagctctcatcccatcggagctgctgcgactcccgcaggttcttccggaactggtttagcttgcccgcaggatcaggaaagtttgagaaaagcatctgcagctgagctgccagttcctctgagtcctcaaagaccaggccattttcttcatgtttcaccagctcatgtaaacacttgaagttcacagcacacacaggcaaacagcacccgaacatgtccaccaccttcatgggcaggtccaggccactggaggacgtgtgcagacagacacccaggtccgccgaccctagaagcagggggtagtcctcggcctccagccagggggtgcagacctggatgtgctggaagtgcttctggtggatgaggcggctataatactccctcagaggccctttgcctgttatcacacagacgagagaaggaaggttgtgtccatcaagagtcagttgttcaaacttttctaaagctgccagcaggatggagaagtcttcgtcctctgtccagctcgtgctgctgaccagcagggctggccgctcacggagacgcgtcaccagcccgctcccagcatcccgctccgtgaaggccgaccgctccgtgactgggtcctcaggttctgagcgggccctgaacggagagtgcatgctgcccagcttcatgaagagccggtgctgcaggtccagaggtgtctctttaaagaaagatgcgggcttgtcgtagacggtcacagccctgatgtgccagttatccgccaggtcttctcgcatagcattggtaacacacaggttcaggtgggacaggcgcccaaagaacttctcgtaccacttggccagcagaacgaggggatggttggggccatgcaccagacccatgatggagtagccatagttgtgccagtcaatgacgagcttgcttccacaaaggcagcccacgaaccagcagacagcaatgctaggcagacctggggggttctggagaaagatataggcacctggctccctccacatcaacttccacagcaagtacatagcctgaagtacaactttgactccgtactggaaaactcggggcccaactgcaagactctgaagttctgtcaaccccacaatctgaattctgttgttctgcaagagctcatcatggggtttggagttaggagaattacgtgagaccacgcaatggattcacttaacacacttctgacacgtg

SEQ ID NO: 15696 - RNA, 2609 nt, Homo sapiens
  source 1..2609: mol_type = other RNA
gctgggattacaggcatgagccactgtgcccggccgctttctaagctttgtgaagagtgggttgactattcagatctctgcttctgtcccgctgtgccaagtgctggggcagacacaggcagagagtggacagcggcacggtgcctgctgctagccatttctatgcaaaaccagctttctggtcccatcctggaggccaattctaggcacctgggtgggcctgggaacctgtgaaccaagtaaactgacttggacacccccctaccccgccaggcctgtcctagcagccccacacaataccctcatgtcctgtccccaaacaccgccatcctcaaacacatgtgctctgtttccaggccgggccgggatcagatgggaagtggaacctcgtcatgagcagaaactgtttccctacgaagagcacttggagatggcaatgctgaatctcaccctgtaggactcacacacgactccaacgggattgtgagaatcaagtcactctcatgggaagaatttttatatgggaaagcggataaaactttcattggactggaatgtttggagaatgttaatttccaaatcaggaaccacaaactgccctctaataagacatcggctatctaagcgtgtgggtgccccctttctgccagcagttctggttcttaagaaaatcaccataaatcagacatgaaaattctggctccaaaaatagcattttctttgtgcaaataaaaacgtgtgtatcaagtatgatgttcccccaacgtggacacactcagttcctcacaaagccaagcccactgcagctgccacatccctgggcttacggtgcagcaggtgcttttttcaagacaggaatcaaaatgttaggaacacggcagaaaggggacacctggagaccaaacgcaggatgaggagttctgcagaggtcacagggaagtcacagaacagtaatacgctagcaggggcatggggcgtgaagaacagaagaagagaggaagcgtttccaagcctccagagaagaaatcaaggccaaccaaagcttcccgggtcacagaaccaattcttttaccaggcagtaccactgctgtcatttcagcttctggccactgggaggtgctgctcgaaagggtttgccctgagactccaagaagaagctgcgggaaggacagcaggggtcctggggttttagcctctggcccaggagttatgtgtccataaccaaagggagcacagtctgcacccagctctcatcccatcggagctgctgcgactcccgcaggttcttccggaactggtttagcttgcccgcaggatcaggaaagtttgagaaaagcatctgcagctgagctgccagttcctctgagtcctcaaagaccaggccattttcttcatgtttcaccagctcatgtaaacacttgaagttcacagcacacacaggcaaacagcacccgaacatgtccaccaccttcatgggcaggtccaggccactggaggacgtgtgcagacagacacccaggtccgccgaccctagaagcagggggtagtcctcggcctccagccagggggtgcagacctggatgtgctggaagtgcttctggtggatgaggcggctataatactccctcagaggccctttgcctgttatcacacagacgagagaaggaaggttgtgtccatcaagagtcagttgttcaaacttttctaaagctgccagcaggatggagaagtcttcgtcctctgtccagctcgtgctgctgaccagcagggctggccgctcacggagacgcgtcaccagcccgctcccagcatcccgctccgtgaaggccgaccgctccgtgactgggtcctcaggttctgagcgggccctgaacggagagtgcatgctgcccagcttcatgaagagccggtgctgcaggtccagaggtgtctctttaaagaaagatgcgggcttgtcgtagacggtcacagccctgatgtgccagttatccgccaggtcttctcgcatagcattggtaacacacaggttcaggtgggacaggcgcccaaagaacttctcgtaccacttggccagcagaacgaggggatggttggggccatgcaccagacccatgatggagtagccatagttgtgccagtcaatgacgagcttgcttccacaaaggcagcccacgaaccagcagacagcaatgctaggcagacctggggggttctggagaaagatataggcacctggctccctccacatcaacttccacagcaagtacatagcctgaagtacaactttgactccgtactggaaaactcggggcccaactgcaagactctgaagttctgtcaaccccacaatctgaattctgttgttctgcaagagctcatcatggggtttggagttgcagaaccccaggagggtcaccgagaagccgtgcatggccaacgacagcgcgtggtactgcatacgggggctgcggcccacgtcgcccagcaccaccgctactacatgccgggccgcccgcccccggcgccagcgcttccatcctcccagcagcagcagcggcagcagcagacacagcgccagcaggaccaagcatgaggccgccatcttggct

SEQ ID NO: 15697 - RNA, 7421 nt, Homo sapiens
  source 1..7421: mol_type = other RNA
gctgggattacaggcatgagccactgtgcccggccggctgtttcttgatagactgctttcctgctgttaaaaataattttatcatactaaaaaacaaaacactacatatttgttataagcagcaatttcagagagaatgaatttggaaagagaaagaaaatgtgacctgagcaatattagttcataggaaagataaaagtaacctaatcagtcacattttgacaattttttaataaacgaatgcagttagtacattctctataattgtccacgtaaaattaaatgcttaataccttttgaagaataaattattagttcccataactagacagttggaattacagcaaaacagtcatccacagaagctctattgtccagcgtttagaaatgtgaatacaaagcaaaccctaacttggcaattacatatatatatttatttataagcatttagctaaaatttatttagtgaataattgaaacatacataatttgccaatataatgtaagcttggatttccatattctaaaacttttgtttttctaaatatttcaaagaaacttatgtctataatttaatatattcaagtatagttcccttttctcttatgtattagcaaccaaactgaattttaggtgatcaagcataacattttattgaaagtatatgatggaattcactacactgtaagactaaaaccaggaacagtgcatccatgagtataatgtatgttgtgaataatcactatcaatgccactatattcccacataaaaaggcaaatagcccactattgatttattctgctaatttcaacaatcattgatcttgaggtacatgccaaaaatgcctgaataagctttgaaatgtaaaacaaaaatgttttaaagaagtttaattgcagttggccaatatatacttaatatggcttgcatttttttttttttttttttgaaataacattgtgacttaaaggatttctaggtcctaaaatctggaaaagggatctggaaaaatttggactccatgagtagtttggattcaatctctctgtgcttttttttttctttataacaggaatgggatggggggtggggggaataaaacttcttatgctatataggtcatgtactgtgagaaacaagaatacaaaactatgggtttaaaaacaacatatacagaaataatcgccaatctctgtctacctccacatcattttgtcatagaagttcattgtgattaaaaagtttaaaagtttttaagagaaaaggtagattgagaagtagaaaggaagtaggaaggaaattgtgcaaaaaaagaaacagtttattagatactctgaccctgggacacactgttcctttcccccaaaatattttccgtgataggaactgaatttaaaattatcaccttgttagattgcctgaagatccagcaactaaaaacttgattaatgcacaacttccttaaaaaatgccaattaactattagccactgacagaaaaatgtaaattaatttaataagatagctttcctttcacctttttagctggaaatgtctgttctgatagaatggatatcctgatttggggaagaggaagaggaaggaacaaggagtaaggatcacacagaatccttctggggatagggtaaatttcgttgatggagtattgctgtgaggtgctcaaataagatagatagcatgaaggggctggaaagccaggagaaagagaatgtacagaataccacaaatatgctttgcccactttaaagcctaagttttcttgtgggccttagggccaagataaatggttgttttccttcttcatatatgaaagacctctatctagaaaatactagtcaatctgtatggaagtttctctgggcagtactattttaacatgttgttccaatgggcagacattataaataccaagcatctgttcttaaggttgtgggttgcctaaacatatggaatccctttgagccaaacagaggtgctatcaaaattgttttattatattgaattaccaatgacaataaattacaaaaaacactgttttagacattgctgagtctaacaaaataggctgaagtttgatctttgtgaaaggacttgaaaccattgttttttcccacaaaaatccccatcaccagcactgcattcgaattttcttgaaaattgtttcctgagtttattcatggtagtatgtgcttaaggacaacaggttgttagtctatttgagcaaacctgatgttttctctaagaaaaacaaattcaatatcctcccccttcaagaacaataaaaccccaaactgtgctatcattaaatactaccaaaaaccattaactagaaaaacacaatgcaaaatcattattcaagaacccattagaaaccacagtattctaaagtcttatagaaaagatgtgtttttactagttaagcattgatagaagtcccatcaaaaaaatgttcaatccaaatctgcatttttggctatggagttctagccaaactggacaggattaggcatccttacctgggctccttctacaaaatgacagtatgttttgaagctctcccatataataaggttgccccctactactgtggttaagctagcatatttgagtttttcactagaaaactctcaaacaattatcgggtacatccagtagcatacctgtatcttttatacactgtcagtcctcactgggtgatcagaaatcatgctgttcattgcttaattcttatagtgttccttttatgataggactgtatggcatgacctttctgagcaagctaatttaaaattaattaagactgtctactttttaaagccattgattatagaaaacctgaaagttattttgtaatcatttttcattttctgatttcacttcccctaattttattacttaaaatgcatccatggaaatagtatctctgtcctgaaaacttcaacaccaaaatcacacctctgagtttgacttatcgattctgataggaaggcataacagcactagataatgacagaaggaaaataagtcagaatatatgcttacaaactgttacatgcaagtacatatagtaataaagcaaatgagaaaaaaagccaaaatggaacataaaaagccataagacatgatacctaactacttctaagtaattatttttcatgtggcataaattgttatttaatctctttcaattatttccaaaagatacctcaaaataagaatacatactttaatatatcacacccaggaaacagatatttgtgcatggggtatagattatttacattacaaacagaatatgtatagtttcttttattaaataccaaagttacgagtttcctagcctaaattgtataattcagcactcagtaatcaactttctctctgaataaagcaaaataaaatacatagcaaatagtacacctaacacgcacaagtagttcacttatattcactaaagaaaactgtgatatcctccagtttacattcatgaattctttctgtcagtagtagtagtagtagtagtagtagtagtagtagtagcagtagtagctgctgctgttgttgtagcaacggtattttcttcaacaacgtgaaatgattctttagcatttcatcatttagagaaaagaatacatactacacagtggttctgaattatacattaaataagaccaatttggccagttttttataaatatgattttaaaatgtgctcaaattttttgtagaccattaatattattcatatttaaaatgttagtttatcttcatgaagtaaaatgattaagtagcattgtctaaagtttactgtaatacaatatactatatcatgtgtgctatatgcacaagtccactacagcaagatgtcaactgtattatcataggattcaaggtagaatgatatgctacactgtacttcaaagcacatcgaagtcagaaaaacaacagtgtagttcatttataaaggggatagatgatgattacaatccaattggttaacttgaaagtcagtttatataacaccaggatagtgtcaacaccacatacttcattttcaaaggcttaactatgacctatttataagattacaccaacagtataaagcctttggaaaaaaaaaaagtttcacttgtactaaatttccatgatgtaaaatttacagaagccttataaaaacctttatttctaaatgaggccacttattatggataatatacagatctgcctgcacacattatctgagatataattcttctataaaaactttggcaccaactatatcaagaattcatatattagcacaaatgtattttgctctggcaccaaaccactatgtttacattttagtaactacagtgagtcaaatgaatggagtcctttggttttacggaataacaagcttttataataagtttttgttgtttttctttcattagaaaaagcctatccttcaggatctgatgtttaaaaatactaacattgcttgtcattatactattatatatgtatactgattgttggtaatgactccccaaaccataattgtatgaaacaagaaaaaaaatattaaagtaactttatttgaaaggaattttagaagcttgtgtgcagagaagttgtgaggacctggtggacaccaattatatgcttaaataaacacttgaacactactgcaaacacatagtatgaatattgtggacctgtgaatggttttttaaatctcacttcccctaaaaatggggatttaatattacttaatattcaagtaatttagcagacaacgatgcctttgataagaataggaaaaaagccacacatttaatttcatcttcatccagtttggcctaggaacaccacaaatcttacaggccagttgatgttcgctttttcatgctccgtcgctgggctaagcttgaagcagctacaggctctaggactggttgaaaggtcttgtgagtcagggcagagtatgttgcaaccattgctcccttaacaacatgtgacacatcatttctctttggctgatcatttggcaactggtctctgtgagttatccatgagtgctttaatatttgttcagcagtataccgctgatgtgggtccatatgaagcatatgggaaagcaaatcctttgctccgtctgaaatattgtcccagtttccaccactcaaagagaattttccattgcctatacgcagcagtatctcttcaggagtatcattggggccattagcaaatggagtgtagccagccaacattgtgtaaaaaaggactcctaaactccagatatcacaagcagcatcatatccctgttgcataagaacctcaggtgcaacaaagtttgcagtgtagcatggagttaagagaagtccattttctcctcgaagttgttttgcaaacccaaaatcacatatcctgattgaatctgcactggctgattcatccatgtataaaatattactaggtttaagatcacgatgaacaactccttgacaatgaagatagtcaactgtcttacttattacatatagtatatcactagcctcccgttccgagaaacatttttgtttgagaatacggtcaagtaactctcctcctttcattaaatccgtaacaaggtaaacatatctaccatcatcaaagacatccttcaaagtaataatgttgggatgttgtccatagcgcatcaatatttcaatctcttctgaagggtctcgcttacttttgtcaatgatcttcactgcaaattccatgttggtagttgcatgtatgcatcgcttgcaaacagagtaggagccaacaccaatatcctccttcaattcatatacttcaccaaattgtgcagcatttccatttatctgaacaattggtaatacatttgcacttgtgataggagtgattttatattcttctgcaatagaagttgcaacaaagctgaatcctttgaagagctgatgagcatttgcactggctggcaaaccgggagaatctttaggtgtttttgcagtaaattcaggatcaaaacaaaaagtatcatctggttttccagaagcaggtttgaaaggaggttgaacttctcttttatataatttatcccagtcaatatttgcaaaaaacagatgtcttttgatttcttcaactccttctgatcccaatctatttgctggattccttttgaataacatccttagaagactttgtgcttcagcactaagaaattgaggcattccaagttttgcttttaatatcatattcatggtctcatttctgtctttaccttgaaatggcagagtaccagtaagcatttcaaacataagaacaccatatgaccaccaatcagcactctgggaatggcctctcctatttactacttcaggagccatatactctactgtaccacaaaatgagtaagccttcttttcttgatctactgactccttgctgagtccaaaatctgttaatttgatatgtcctatttcatcaagcaaaatgttttctggcttcaggtctctataaacaattcctaattggtgcagatgatccaaagcaagggccagttctgcgaggtagaatttcacatcttcctctgtaaacagaacctctttggataatcttgtgaaaacatctcctcccctgagaaaatccagtattaagtacagtttcccttcagtctgaaaggcatagtgcaatttgacaataaatggatgatttacttccaccagtatatccctctccatctttgtccgaactctgtctcgaacttttaaagaggctttttttaacaccttcattgcatagagctgcccagcatcaggaccggtcttctttctaacaagaaaaacctttccaaatgacccctgaccaagaaccttgagcaactcaaactgtgcaggatctgctttctcatagccttccttaacatgatgagtaatagggatttctttaacaactccttcatcatgacaagaatctgcttctccctcttccattggctcatcaaccattttaagaccatttacctcgccgctgctcgcgccgccgccgctgaacacttccatttctcggtcccagggctcgtcctgaggagcgaatggtagcatctccccttcaggagcactcaaacaggagctgccgcctaccgctggcgcggccgcgcatcctgtctattgaactggcccgccgccgccgccgccgccgccgccgccgccgcgacccccagccccgccttcagcgagcgctgccctcgccgccgggtctctcagaggctgggagctgggggtcgccgccgccgccgcccggtgattcccatagagaagacaactctgtgctgcctctccaagagctgccgctcggctcgcgctcaccactgccaccacaacgacagccgctcggtggtgact

SEQ ID NO: 15698 - RNA, 7379 nt, Homo sapiens
  source 1..7379: mol_type = other RNA
gctgggattacaggcatgagccactgtgcccggccggctgtttcttgatagactgctttcctgctgttaaaaataattttatcatactaaaaaacaaaacactacatatttgttataagcagcaatttcagagagaatgaatttggaaagagaaagaaaatgtgacctgagcaatattagttcataggaaagataaaagtaacctaatcagtcacattttgacaattttttaataaacgaatgcagttagtacattctctataattgtccacgtaaaattaaatgcttaataccttttgaagaataaattattagttcccataactagacagttggaattacagcaaaacagtcatccacagaagctctattgtccagcgtttagaaatgtgaatacaaagcaaaccctaacttggcaattacatatatatatttatttataagcatttagctaaaatttatttagtgaataattgaaacatacataatttgccaatataatgtaagcttggatttccatattctaaaacttttgtttttctaaatatttcaaagaaacttatgtctataatttaatatattcaagtatagttcccttttctcttatgtattagcaaccaaactgaattttaggtgatcaagcataacattttattgaaagtatatgatggaattcactacactgtaagactaaaaccaggaacagtgcatccatgagtataatgtatgttgtgaataatcactatcaatgccactatattcccacataaaaaggcaaatagcccactattgatttattctgctaatttcaacaatcattgatcttgaggtacatgccaaaaatgcctgaataagctttgaaatgtaaaacaaaaatgttttaaagaagtttaattgcagttggccaatatatacttaatatggcttgcatttttttttttttttttttgaaataacattgtgacttaaaggatttctaggtcctaaaatctggaaaagggatctggaaaaatttggactccatgagtagtttggattcaatctctctgtgcttttttttttctttataacaggaatgggatggggggtggggggaataaaacttcttatgctatataggtcatgtactgtgagaaacaagaatacaaaactatgggtttaaaaacaacatatacagaaataatcgccaatctctgtctacctccacatcattttgtcatagaagttcattgtgattaaaaagtttaaaagtttttaagagaaaaggtagattgagaagtagaaaggaagtaggaaggaaattgtgcaaaaaaagaaacagtttattagatactctgaccctgggacacactgttcctttcccccaaaatattttccgtgataggaactgaatttaaaattatcaccttgttagattgcctgaagatccagcaactaaaaacttgattaatgcacaacttccttaaaaaatgccaattaactattagccactgacagaaaaatgtaaattaatttaataagatagctttcctttcacctttttagctggaaatgtctgttctgatagaatggatatcctgatttggggaagaggaagaggaaggaacaaggagtaaggatcacacagaatccttctggggatagggtaaatttcgttgatggagtattgctgtgaggtgctcaaataagatagatagcatgaaggggctggaaagccaggagaaagagaatgtacagaataccacaaatatgctttgcccactttaaagcctaagttttcttgtgggccttagggccaagataaatggttgttttccttcttcatatatgaaagacctctatctagaaaatactagtcaatctgtatggaagtttctctgggcagtactattttaacatgttgttccaatgggcagacattataaataccaagcatctgttcttaaggttgtgggttgcctaaacatatggaatccctttgagccaaacagaggtgctatcaaaattgttttattatattgaattaccaatgacaataaattacaaaaaacactgttttagacattgctgagtctaacaaaataggctgaagtttgatctttgtgaaaggacttgaaaccattgttttttcccacaaaaatccccatcaccagcactgcattcgaattttcttgaaaattgtttcctgagtttattcatggtagtatgtgcttaaggacaacaggttgttagtctatttgagcaaacctgatgttttctctaagaaaaacaaattcaatatcctcccccttcaagaacaataaaaccccaaactgtgctatcattaaatactaccaaaaaccattaactagaaaaacacaatgcaaaatcattattcaagaacccattagaaaccacagtattctaaagtcttatagaaaagatgtgtttttactagttaagcattgatagaagtcccatcaaaaaaatgttcaatccaaatctgcatttttggctatggagttctagccaaactggacaggattaggcatccttacctgggctccttctacaaaatgacagtatgttttgaagctctcccatataataaggttgccccctactactgtggttaagctagcatatttgagtttttcactagaaaactctcaaacaattatcgggtacatccagtagcatacctgtatcttttatacactgtcagtcctcactgggtgatcagaaatcatgctgttcattgcttaattcttatagtgttccttttatgataggactgtatggcatgacctttctgagcaagctaatttaaaattaattaagactgtctactttttaaagccattgattatagaaaacctgaaagttattttgtaatcatttttcattttctgatttcacttcccctaattttattacttaaaatgcatccatggaaatagtatctctgtcctgaaaacttcaacaccaaaatcacacctctgagtttgacttatcgattctgataggaaggcataacagcactagataatgacagaaggaaaataagtcagaatatatgcttacaaactgttacatgcaagtacatatagtaataaagcaaatgagaaaaaaagccaaaatggaacataaaaagccataagacatgatacctaactacttctaagtaattatttttcatgtggcataaattgttatttaatctctttcaattatttccaaaagatacctcaaaataagaatacatactttaatatatcacacccaggaaacagatatttgtgcatggggtatagattatttacattacaaacagaatatgtatagtttcttttattaaataccaaagttacgagtttcctagcctaaattgtataattcagcactcagtaatcaactttctctctgaataaagcaaaataaaatacatagcaaatagtacacctaacacgcacaagtagttcacttatattcactaaagaaaactgtgatatcctccagtttacattcatgaattctttctgtcagtagtagtagtagtagtagtagtagtagtagtagtagcagtagtagctgctgctgttgttgtagcaacggtattttcttcaacaacgtgaaatgattctttagcatttcatcatttagagaaaagaatacatactacacagtggttctgaattatacattaaataagaccaatttggccagttttttataaatatgattttaaaatgtgctcaaattttttgtagaccattaatattattcatatttaaaatgttagtttatcttcatgaagtaaaatgattaagtagcattgtctaaagtttactgtaatacaatatactatatcatgtgtgctatatgcacaagtccactacagcaagatgtcaactgtattatcataggattcaaggtagaatgatatgctacactgtacttcaaagcacatcgaagtcagaaaaacaacagtgtagttcatttataaaggggatagatgatgattacaatccaattggttaacttgaaagtcagtttatataacaccaggatagtgtcaacaccacatacttcattttcaaaggcttaactatgacctatttataagattacaccaacagtataaagcctttggaaaaaaaaaaagtttcacttgtactaaatttccatgatgtaaaatttacagaagccttataaaaacctttatttctaaatgaggccacttattatggataatatacagatctgcctgcacacattatctgagatataattcttctataaaaactttggcaccaactatatcaagaattcatatattagcacaaatgtattttgctctggcaccaaaccactatgtttacattttagtaactacagtgagtcaaatgaatggagtcctttggttttacggaataacaagcttttataataagtttttgttgtttttctttcattagaaaaagcctatccttcaggatctgatgtttaaaaatactaacattgcttgtcattatactattatatatgtatactgattgttggtaatgactccccaaaccataattgtatgaaacaagaaaaaaaatattaaagtaactttatttgaaaggaattttagaagcttgtgtgcagagaagttgtgaggacctggtggacaccaattatatgcttaaataaacacttgaacactactgcaaacacatagtatgaatattgtggacctgtgaatggttttttaaatctcacttcccctaaaaatggggatttaatattacttaatattcaagtaatttagcagacaacgatgcctttgataagaataggaaaaaagccacacatttaatttcatcttcatccagtttggcctaggaacaccacaaatcttacaggccagttgatgttcgctttttcatgctccgtcgctgggctaagcttgaagcagctacaggctctaggactggttgaaaggtcttgtgagtcagggcagagtatgttgcaaccattgctcccttaacaacatgtgacacatcatttctctttggctgatcatttggcaactggtctctgtgagttatccatgagtgctttaatatttgttcagcagtataccgctgatgtgggtccatatgaagcatatgggaaagcaaatcctttgctccgtctgaaatattgtcccagtttccaccactcaaagagaattttccattgcctatacgcagcagtatctcttcaggagtatcattggggccattagcaaatggagtgtagccagccaacattgtgtaaaaaaggactcctaaactccagatatcacaagcagcatcatatccctgttgcataagaacctcaggtgcaacaaagtttgcagtgtagcatggagttaagagaagtccattttctcctcgaagttgttttgcaaacccaaaatcacatatcctgattgaatctgcactggctgattcatccatgtataaaatattactaggtttaagatcacgatgaacaactccttgacaatgaagatagtcaactgtcttacttattacatatagtatatcactagcctcccgttccgagaaacatttttgtttgagaatacggtcaagtaactctcctcctttcattaaatccgtaacaaggtaaacatatctaccatcatcaaagacatccttcaaagtaataatgttgggatgttgtccatagcgcatcaatatttcaatctcttctgaagggtctcgcttacttttgtcaatgatcttcactgcaaattccatgttggtagttgcatgtatgcatcgcttgcaaacagagtaggagccaacaccaatatcctccttcaattcatatacttcaccaaattgtgcagcatttccatttatctgaacaattggtaatacatttgcacttgtgataggagtgattttatattcttctgcaatagaagttgcaacaaagctgaatcctttgaagagctgatgagcatttgcactggctggcaaaccgggagaatctttaggtgtttttgcagtaaattcaggatcaaaacaaaaagtatcatctggttttccagaagcaggtttgaaaggaggttgaacttctcttttatataatttatcccagtcaatatttgcaaaaaacagatgtcttttgatttcttcaactccttctgatcccaatctatttgctggattccttttgaataacatccttagaagactttgtgcttcagcactaagaaattgaggcattccaagttttgcttttaatatcatattcatggtctcatttctgtctttaccttgaaatggcagagtaccagtaagcatttcaaacataagaacaccatatgaccaccaatcagcactctgggaatggcctctcctatttactacttcaggagccatatactctactgtaccacaaaatgagtaagccttcttttcttgatctactgactccttgctgagtccaaaatctgttaatttgatatgtcctatttcatcaagcaaaatgttttctggcttcaggtctctataaacaattcctaattggtgcagatgatccaaagcaagggccagttctgcgaggtagaatttcacatcttcctctgtaaacagaacctctttggataatcttgtgaaaacatctcctcccctgagaaaatccagtattaagtacagtttcccttcagtctgaaaggcatagtgcaatttgacaataaatggatgatttacttccaccagtatatccctctccatctttgtccgaactctgtctcgaacttttaaagaggctttttttaacaccttcattgcatagagctgcccagcatcaggaccggtcttctttctaacaagaaaaacctttccaaatgacccctgaccaagaaccttgagcaactcaaactgtgcaggatctgctttctcatagccttccttaacatgatgagtaatagggatttctttaacaactccttcatcatgacaagaatctgcttctccctcttccattggctcatcaaccattttaagaccatttaccttcacctttcgttttacttcatagggattaacaatttccactcgagtatttttccaaattgctgaggtagagagacccattgttaaatctctacaatacctaaaacatactcaaaatatcctactgtgaatcaatttcaccaactatttttaggaggtgtatggtggcctctactggagtagtacgcagtcgattaagttatcagaaaaggatccaactttctcgccgctgctcgcgccgccgccgctgaacacttccatttctcggtcccagggctcgtcctgaggagcgaatggtagcatctccccttcaggagcactcaaacaggagctgccgcc

SEQ ID NO: 15699 - RNA, 8327 nt, Homo sapiens
  source 1..8327: mol_type = other RNA
gctgggattacaggcatgagccactgtgcccggccggctgtttcttgatagactgctttcctgctgttaaaaataattttatcatactaaaaaacaaaacactacatatttgttataagcagcaatttcagagagaatgaatttggaaagagaaagaaaatgtgacctgagcaatattagttcataggaaagataaaagtaacctaatcagtcacattttgacaattttttaataaacgaatgcagttagtacattctctataattgtccacgtaaaattaaatgcttaataccttttgaagaataaattattagttcccataactagacagttggaattacagcaaaacagtcatccacagaagctctattgtccagcgtttagaaatgtgaatacaaagcaaaccctaacttggcaattacatatatatatttatttataagcatttagctaaaatttatttagtgaataattgaaacatacataatttgccaatataatgtaagcttggatttccatattctaaaacttttgtttttctaaatatttcaaagaaacttatgtctataatttaatatattcaagtatagttcccttttctcttatgtattagcaaccaaactgaattttaggtgatcaagcataacattttattgaaagtatatgatggaattcactacactgtaagactaaaaccaggaacagtgcatccatgagtataatgtatgttgtgaataatcactatcaatgccactatattcccacataaaaaggcaaatagcccactattgatttattctgctaatttcaacaatcattgatcttgaggtacatgccaaaaatgcctgaataagctttgaaatgtaaaacaaaaatgttttaaagaagtttaattgcagttggccaatatatacttaatatggcttgcatttttttttttttttttttgaaataacattgtgacttaaaggatttctaggtcctaaaatctggaaaagggatctggaaaaatttggactccatgagtagtttggattcaatctctctgtgcttttttttttctttataacaggaatgggatggggggtggggggaataaaacttcttatgctatataggtcatgtactgtgagaaacaagaatacaaaactatgggtttaaaaacaacatatacagaaataatcgccaatctctgtctacctccacatcattttgtcatagaagttcattgtgattaaaaagtttaaaagtttttaagagaaaaggtagattgagaagtagaaaggaagtaggaaggaaattgtgcaaaaaaagaaacagtttattagatactctgaccctgggacacactgttcctttcccccaaaatattttccgtgataggaactgaatttaaaattatcaccttgttagattgcctgaagatccagcaactaaaaacttgattaatgcacaacttccttaaaaaatgccaattaactattagccactgacagaaaaatgtaaattaatttaataagatagctttcctttcacctttttagctggaaatgtctgttctgatagaatggatatcctgatttggggaagaggaagaggaaggaacaaggagtaaggatcacacagaatccttctggggatagggtaaatttcgttgatggagtattgctgtgaggtgctcaaataagatagatagcatgaaggggctggaaagccaggagaaagagaatgtacagaataccacaaatatgctttgcccactttaaagcctaagttttcttgtgggccttagggccaagataaatggttgttttccttcttcatatatgaaagacctctatctagaaaatactagtcaatctgtatggaagtttctctgggcagtactattttaacatgttgttccaatgggcagacattataaataccaagcatctgttcttaaggttgtgggttgcctaaacatatggaatccctttgagccaaacagaggtgctatcaaaattgttttattatattgaattaccaatgacaataaattacaaaaaacactgttttagacattgctgagtctaacaaaataggctgaagtttgatctttgtgaaaggacttgaaaccattgttttttcccacaaaaatccccatcaccagcactgcattcgaattttcttgaaaattgtttcctgagtttattcatggtagtatgtgcttaaggacaacaggttgttagtctatttgagcaaacctgatgttttctctaagaaaaacaaattcaatatcctcccccttcaagaacaataaaaccccaaactgtgctatcattaaatactaccaaaaaccattaactagaaaaacacaatgcaaaatcattattcaagaacccattagaaaccacagtattctaaagtcttatagaaaagatgtgtttttactagttaagcattgatagaagtcccatcaaaaaaatgttcaatccaaatctgcatttttggctatggagttctagccaaactggacaggattaggcatccttacctgggctccttctacaaaatgacagtatgttttgaagctctcccatataataaggttgccccctactactgtggttaagctagcatatttgagtttttcactagaaaactctcaaacaattatcgggtacatccagtagcatacctgtatcttttatacactgtcagtcctcactgggtgatcagaaatcatgctgttcattgcttaattcttatagtgttccttttatgataggactgtatggcatgacctttctgagcaagctaatttaaaattaattaagactgtctactttttaaagccattgattatagaaaacctgaaagttattttgtaatcatttttcattttctgatttcacttcccctaattttattacttaaaatgcatccatggaaatagtatctctgtcctgaaaacttcaacaccaaaatcacacctctgagtttgacttatcgattctgataggaaggcataacagcactagataatgacagaaggaaaataagtcagaatatatgcttacaaactgttacatgcaagtacatatagtaataaagcaaatgagaaaaaaagccaaaatggaacataaaaagccataagacatgatacctaactacttctaagtaattatttttcatgtggcataaattgttatttaatctctttcaattatttccaaaagatacctcaaaataagaatacatactttaatatatcacacccaggaaacagatatttgtgcatggggtatagattatttacattacaaacagaatatgtatagtttcttttattaaataccaaagttacgagtttcctagcctaaattgtataattcagcactcagtaatcaactttctctctgaataaagcaaaataaaatacatagcaaatagtacacctaacacgcacaagtagttcacttatattcactaaagaaaactgtgatatcctccagtttacattcatgaattctttctgtcagtagtagtagtagtagtagtagtagtagtagtagtagcagtagtagctgctgctgttgttgtagcaacggtattttcttcaacaacgtgaaatgattctttagcatttcatcatttagagaaaagaatacatactacacagtggttctgaattatacattaaataagaccaatttggccagttttttataaatatgattttaaaatgtgctcaaattttttgtagaccattaatattattcatatttaaaatgttagtttatcttcatgaagtaaaatgattaagtagcattgtctaaagtttactgtaatacaatatactatatcatgtgtgctatatgcacaagtccactacagcaagatgtcaactgtattatcataggattcaaggtagaatgatatgctacactgtacttcaaagcacatcgaagtcagaaaaacaacagtgtagttcatttataaaggggatagatgatgattacaatccaattggttaacttgaaagtcagtttatataacaccaggatagtgtcaacaccacatacttcattttcaaaggcttaactatgacctatttataagattacaccaacagtataaagcctttggaaaaaaaaaaagtttcacttgtactaaatttccatgatgtaaaatttacagaagccttataaaaacctttatttctaaatgaggccacttattatggataatatacagatctgcctgcacacattatctgagatataattcttctataaaaactttggcaccaactatatcaagaattcatatattagcacaaatgtattttgctctggcaccaaaccactatgtttacattttagtaactacagtgagtcaaatgaatggagtcctttggttttacggaataacaagcttttataataagtttttgttgtttttctttcattagaaaaagcctatccttcaggatctgatgtttaaaaatactaacattgcttgtcattatactattatatatgtatactgattgttggtaatgactccccaaaccataattgtatgaaacaagaaaaaaaatattaaagtaactttatttgaaaggaattttagaagcttgtgtgcagagaagttgtgaggacctggtggacaccaattatatgcttaaataaacacttgaacactactgcaaacacatagtatgaatattgtggacctgtgaatggttttttaaatctcacttcccctaaaaatggggatttaatattacttaatattcaagtaatttagcagacaacgatgcctttgataagaataggaaaaaagccacacatttaatttcatcttcatccagtttggcctaggaacaccacaaatcttacaggccagttgatgttcgctttttcatgctccgtcgctgggctaagcttgaagcagctacaggctctaggactggttgaaaggtcttgtgagtcagggcagagtatgttgcaaccattgctcccttaacaacatgtgacacatcatttctctttggctgatcatttggcaactggtctctgtgagttatccatgagtgctttaatatttgttcagcagtataccgctgatgtgggtccatatgaagcatatgggaaagcaaatcctttgctccgtctgaaatattgtcccagtttccaccactcaaagagaattttccattgcctatacgcagcagtatctcttcaggagtatcattggggccattagcaaatggagtgtagccagccaacattgtgtaaaaaaggactcctaaactccagatatcacaagcagcatcatatccctgttgcataagaacctcaggtgcaacaaagtttgcagtgtagcatggagttaagagaagtccattttctcctcgaagttgttttgcaaacccaaaatcacatatcctgattgaatctgcactggctgattcatccatgtataaaatattactaggtttaagatcacgatgaacaactccttgacaatgaagatagtcaactgtcttacttattacatatagtatatcactagcctcccgttccgagaaacatttttgtttgagaatacggtcaagtaactctcctcctttcattaaatccgtaacaaggtaaacatatctaccatcatcaaagacatccttcaaagtaataatgttgggatgttgtccatagcgcatcaatatttcaatctcttctgaagggtctcgcttacttttgtcaatgatcttcactgcaaattccatgttggtagttgcatgtatgcatcgcttgcaaacagagtaggagccaacaccaatatcctccttcaattcatatacttcaccaaattgtgcagcatttccatttatctgaacaattggtaatacatttgcacttgtgataggagtgattttatattcttctgcaatagaagttgcaacaaagctgaatcctttgaagagctgatgagcatttgcactggctggcaaaccgggagaatctttaggtgtttttgcagtaaattcaggatcaaaacaaaaagtatcatctggttttccagaagcaggtttgaaaggaggttgaacttctcttttatataatttatcccagtcaatatttgcaaaaaacagatgtcttttgatttcttcaactccttctgatcccaatctatttgctggattccttttgaataacatccttagaagactttgtgcttcagcactaagaaattgaggcattccaagttttgcttttaatatcatattcatggtctcatttctgtctttaccttgaaatggcagagtaccagtaagcatttcaaacataagaacaccatatgaccaccaatcagcactctgggaatggcctctcctatttactacttcaggagccatatactctactgtaccacaaaatgagtaagccttcttttcttgatctactgactccttgctgagtccaaaatctgttaatttgatatgtcctatttcatcaagcaaaatgttttctggcttcaggtctctataaacaattcctaattggtgcagatgatccaaagcaagggccagttctgcgaggtagaatttcacatcttcctctgtaaacagaacctctttggataatcttgtgaaaacatctcctcccctgagaaaatccagtattaagtacagtttcccttcagtctgaaaggcatagtgcaatttgacaataaatggatgatttacttccaccagtatatccctctccatctttgtccgaactctgtctcgaacttttaaagaggctttttttaacaccttcattgcatagagctgcccagcatcaggaccggtcttctttctaacaagaaaaacctttccaaatgacccctgaccaagaaccttgagcaactcaaactgtgcaggatctgctttctcatagccttccttaacatgatgagtaatagggatttctttaacaactccttcatcatgacaagaatctgcttctccctcttccattggctcatcaaccattttaagaccatttaccttcacctttcgttttacttcatagggattaacaatttccactcgagtatttttccaaattgctgaggtagagagacccattgttaaatctctacaatacctaaaacatactgcaaacaataaaaaaaccatatgtggtaattacaatttaaaacatactacattcaaagttaacagaaataataaaatagtaggcatgcaaaaggattcccacctcccatcccatccttatatcaaagcatttaactgtttttataaactaaatgcctataagttcagtaagttacatacatgaatataacaaagttcctctccccttcaatagacttgctagacaattgtgcaaacagttagcattcccacatttcaacaagaaaggaacgcctattcatttatcttgttcttacgagatgtaaaatattaaaacgtatattggaattgcttggtttactagtaaaatatttcctgtaagtatagagggttcagatttagggtacttctgaatttatttccactatattccttaccacatgttattctagcatgtaatcttaaccccagtttagttgataaataacaaaaaaatttaaagaaaaaaaaacaaggtaatcatacaacagccaaatgtgtattttttttaaatggagcaagtacttgaagacaaagttgcaccctttagatgtcgaggattgagagtcttacctcaaaatatcctactgtgaatcaatttcaccaactatttttaggaggtgtatggtggcctctactggagtagtacgcagtcgattaagttatcagaaaaggatccaactttctatcacaaaagacacgtttttgtgtttaaatgctgcccgcttttataacaacaataaaaacaaagcacctgtgtacatctaagttctcactgcacagctgaccaaagcccaaccagaacagtttcagagtaagaagagtgggaagagaggtgaaccaaagtattttggttgaacctcgctaagtcttaccaaagattcgacttatttataagggctggggtttactttgcgtcttcttttacagaccaacggggcagggacagcggttgtggaaaggagaaggggtggagcaagagtgcagtagaatcaaggggacctgagaggaagcagtagaacatcacctgaaacctggcgactggagataggtcgccagtgtatctcgacatgggtcattacaaggaaccataacaagccacagagaaacgagaaagctgttaccagggaacactcgtgcctatgtgcaaatgtcccc

SEQ ID NO: 15700 - RNA, 4426 nt, Homo sapiens
  source 1..4426: mol_type = other RNA
gctgggattacaggcatgagccactgtgcccggcctaattttcgtatttttagtagagagggggtttcaccatgttggtcaggatggtctcgatctactgaccttgtgatctgcccgcctcggcctcccaaagtgctgggaatacaggtgtgagccaccatgcgcagcctgctgttactttcagtggcaaaaccacaattacttctgcacctaccttgtaggggtgttgcttaacacttattgagattgtgcatataaaggagttagcattgttcagataataaatctcggttgtcatcatcattattgtcatcatgctgatacccagtaagtgaatccatgcaatctaaatccttcatccttttctccagttctagcccagggtcccttggccagaacacatggtcaattgtaaacttgagaggatgtactgggacactttgtaggttttgtaggttgctgacatttcttaaactaactgcatttgttttctagcaatgttgcaacaaagtaccacaaatcaggccgagtgtggtggtttacacctgcaatcccagcactttgtgaagccgaggagggcagatctcttgaggccgggagtttgagaccagcctgggcaacatagtgagaccctgtctctacaaatatatatagctgattgcagtggcataggcctgtagtcccaactactcaggaggctgaggcaggaggattgcttgagcccaggagtttgaggtgaggttgcactttagctatgattgcaccactgtactccagcctgggtgacacagtagatcctgtctgtctctaaaagaaaaaaaaatttaaaaattaccatgaactaggtgacttaaacaatagaaatttgttgtcttacagttctggaggttaagagtccgagatcaaggtgttgggccaggtgcagtggcccacgcttgtaatcccagcactttgggaggctgaggtgggcagatcactggaggccaggagtttgagaccagtctggccaacatagtgaaatcccatctctactaaaaacacaaaattagctgggcgtggtggtgggtgcctgtaatcccagctacttgggaggctgaggcaggagaattgcttgaacctgggaggtggaggttgcagtgagccaaaatcatgccactgcatccagccgggatgacagagcaagactccgtctcaaaaaaaaaaaaaaaaaaaaaagatcagttgtcagcagctttgattccttggttccttctgagggctgagagggatagcctgttccacgcctctcctggcttctggtggtctgcaggcagtccctggcattccttggcttgtaggagcatcaccccaatctctgcctccatcttcatgtggcggtctccatgtgtgtgggtgcctgtgtccaaatctccccttttcataaggacgccagtcgtatcagattagggaccaacctaatgaccttactgtaatctaatgacctctgtaaacaccctatcttcaaatatggtcacattctgaggtccttggggttaggacttcaacatatcttttttattttattattattacttttgcagacagggccttgctctgtttcccaggctggagtgcagtggcaggaacatagctcatgcagcctcgacctccttggctcaagaggtcctcctgtctcagcctcccgagtaactaagatgacaggtgcacaccaccacacccaggtaattttttcttttttcatttttattttttgtagggatgagatctcactatgttgttcaggctggtcctgaactcctagcttcaaatgattctccctactcaacctcccaaagtgccagagtttacaggtgtgagccactgcgcctggcctcccacgtatctttttttgggagccacagttcaacccataacactaactttttaagtgccccgggccacctgatctgctgtggctgaccctgcgtgtagaatcatactgggttcagagtcaggcgatgaatgtcacaggaaacacatagattttggagctaggctagggtctgtgttcccaaactacgattgatggaccgtctgcatcagagtccccttgactgggggttgtggggagacaggaagcctgttgggaattgagaaagtaagccccaaccacagtcatagttacaagtggaggtctcaagaccccccaggaggctgaggcttgctggctgactaagcgaacagcacgtgagctaatctcacttgcaaatattttcaaagttcttccacaacacttaggaaacactggctaatacatgggctgtctgtatctacctatctatctatctatctatctacctacctcctctatctctatctatccatccatctatctatcatctatctgttgatcgattgatcaatcgatcgactgacctacctacctatctcatctatctatctatctatctatctatctatcatctatctacttatatgatctatctatcaatcaatcatctatctgtctgtcaatagatagatctatcgatcggttgacctacctacctacctacctatctatcctatctatctatgtatctatctgtatatctatctatctatctatctatctatctatctatctatctatctatctacatatcttatctatccaccctatctacctatcttatcttatcctctctatctatctgtctgtctatctatctatctatctatctatctatctatctatctatctatctacctatgagtgacagatcttgctcagtttcccaaactgctgaagtgcagtggtgcagtcatagctcactgcaaccttgaactcctgggctcaaatgatctgcctgcctcagcctcctgattagctgagactacaggcgtataccaccatgtcttgctaaagtgattttgtgtgtgtgtgtggagatagggtctctgtatgttgcccaggctggtctcaaactcctggcctcaagtgatccttccaccttggcctcccaaaatgctgggatcacaggcttgagcttccacacctggcctttgtcaatactaaaatgagtgtagctacgtctcttgttttcaactactcttattcacatagcaatcctaaaaggctgatcctccaggagggctaatttcaggccagtttgatccttgctattctgatctttttggggaagataaatcctggggaaaatgcacacctttcctttgggtgctcatacactttgttcatctctttatgacacatttatcacgttgtactggaaggatttattccatgtctctgttcccagctagactctgaactcctccagggtaggggatgggatgcatctctgtgtccctagcagccaacagtgatcctggaacatgataaacatccaataactgttctggcctaggacaggggacggccactttgccgatgagcttccccagggctgccttcatatccttgttccgtatgctgtagataaaggggttgagcatggggatgaacaccccacacattagggcggctgccttgtccttctgggaggagctgggggatgtgggctgtaagtacacagcaaagatggtcccataggacagtgacaccacagtgaggtgtaagccacaggtggagaaggctttccacttgccccgagtagaagggatcttaaagactgtccagaaaatgcggatgtacgagagaaggatgcaggagaatgggctggtgcccacgacaatgccaaaagcaaagatcaccagctcgttggtgtgcgtgtctgagccggagagcttcagcaggggcatgaggtcacagaagaagtgggagatttcagagccggcgcagaaggtcagttgagccatgaggcaggtgtgtatgagagactggaggttggtgatcatccatgatgctcccagcagcagcccacagacaggggagcacatgagaaccaagtaacgctgtgggtggacaatggccacgaagcggtcgatggccattactgccaggagaaagctgtccatggtcccgaacaggtggaaggcatacatctgggtgaggcagcccacaaaggggatggctctgctctgagcctggatgttcgctagcatcttggggacggtggtggaggataatagggtgtcaacgagtgagaggttgaagagaaagaagtacatgggtgtgtggaggtgagagtccgtgatgatggccaggataatgagggcatttccaatgatggtgaccaggtatgtggagaggaacattgtgaagaggagggtctgatgctctggcttttctgagagtccctggaggaagaattctgagatttcggtttgcttttctggttccatgtatggtctgtgactgtgatcgctggggttagcctgatgtctatgggaaggattcatatgtgtacccccccgcccccag

SEQ ID NO: 15701 - RNA, 3659 nt, Homo sapiens
  source 1..3659: mol_type = other RNA
gctgggattacaggcatgagccactgtgcccggcctaccttctattttcactactgtgttaagcatgaaagaaaatccaactgggttagatacagcaggttctcctaaatgtcttaacccatgtttatcttgttctgctattccatgagcaaagagaataaacacaaagctgtgagagtattaaatatggacactagatttacatttccaacaagaaattcatctccctccaaagtcccagaccagggctagaatgtggttcatttttaacaatcaaagtggcaagatctgtttggtgatcactgtaaaaacaggaaacatagctaatgccctttcatgttgaggtgctacaaaggtccaagcttttaaagactatggcctcaacgtccatgtgtgaaacaagtgtattagaaaattctttaagtcttgttgccttaacttagagatctccaggcaacaggcctgacgatagccatggctgtaccacttaactatgattctattccaactgttcagaatcatatcacaaaatgacttgtacacagtagtttacaacgactcccaagagaggaaaaaaaaaaaaagacgcctcaaaattcactcaacttttgagacagcaatggcaataggcagcagagaagctatgctgcaactgagggcacatatcattgaagatgtcacaggagtttaagagacaggctggaaaaaatctcatactaagcaaacagtagtatctcataccaagcaaaaccaagtagtatctgctcagcctgccgctaacagatctcacaatcaccaactgtgctttaggactgtcaccaaagtcagattcggtgctaaccaggtggcatctatgatcaacgtcgcccctcttatttaacaaagggctctgaaggaggtgttctccaagcaacaaggagactgcttcagtacaagactttgcaccttgaattcaattgcatcaagtgtggatagcaaaataagtatcttaccattgaaatatgtgttcagcctaagattttacccaccagcagaacaaaagtgagggtgagagggatgggccagtgaggggatgggggagaaaaaaaaatcacaggattaccaccaaagccttgttttaaaagggctcccttcactattcaggaagggaagtggaaggagaaattaaccaattcctgccacagcagccctttttggctgcttccacaatagatactttatggagtggcacagccaaccctatctgtgacctgccctgcggataaacacagccaagcaggtttaattagatcaaagacacaaagggctattccctcctttcataacaacgcagctgtaagtgcctacaacagcaggggagaaacaaaggcagcagaacagaaccttaattgaaaccttcccctggctggcccttgacaatgatttacttgtaacctaggaaggggcgggtggagcaggaggtagcaggagcctcagctaagagccagctccagaaggctaattacttgggggttgtggaggagggaggtagcaaagtctttgtttgtagcccgagtttgcttaactatttgttacacttaataggaggctgctgtggttttggtctgctgctcccggaccttgtcatggattcaccagccctgcgctccaggaatcccataaaataaatcaccccagcctcctggatcccatacacagctcagctccgccaaagcagacaagcagctttcgtgctggtcccgcagtggcgactccacaaacccactctggcctttctaccaggattcttccaagcccaggataggaagcaacggcaggaatgggtactccgaactttcccccaaccccacgtgcttaagaatggccgattataaacccagatctaccaaggtttaagtgccaggcaagtccacagtttgctccaccgcggagaggaagacagacagggggccagagggagacgccccccacccccaactaaagtgtttcctacctgctccctctgtccccttcctcctcccccgtccacagccggctgcgcatttcaccaactcttttccaaagggcccaggaatcccagatggggcccagacagtggcaaaagagggaggaagagagggagaaagggagcagcggctgctactgcaaacagttccccttcgcagctctgcgctcagctcgcccatcagtgtgccactgcctctccgtcctcctcctcggagctgggcgcaggggggcgcccgggaggcggcgtagtccgcgccacgttgctgtcgccctcctccggctccgccgggtgcaggtgcgtggcgagctcctgcagcacggccgcgcgcccgatctggtcgttgcgtcgcttctccatgatcaggtcctctagactctggaactcgagcgtgtggctgcgctgcgccgacagctgaatctgcagccggtagggctgcttgccgatgcgcagctcgccgccgatcttgaactcgcgcttgccgtagcggcaccaggcggcgaaactctccgagttgcgccagctcagctcgcgctccttggcacccacgtgcgccagcgcgttgcgcaccacggcgctggagcttagcggcttgtagcggtacagatcgttgaccacgcggccgcgacggccctggctggcgtcagtcaggaagctgttaatcacctccagccggtgcaggtgcaccacctggaagttacccacatatacggcccagtgcgggtactgagcctgcgacacgaactccaccagatcgcccggcttgcacttgttgagcaggttctcgggcgtgtaggtactcagcgccgccgagcccggcgcgaagctcttctggtagatgcattcgtcccggtagaacacggagcattccacctcgtgcagccgcggatcgtagggctgcggctggggcggcggcggcccgtccccaccgtcgggcaagccgccgccatctggcccctgaggcggcggctgcggctccacgtcctcatcgtcattggagaaaatgtaggagaccccaatgcggggcccgtcgtcccggtccacgccagtcgggtcggccgtgggaacttccttgtaacttaggtgggtcaatttctccacctggttgcccatcacgctgcggacacacgttcacaccgccgcaaggggagaaagcgaaaccaactccagggtcatttgcacaggtccccggacaggggctgaggctacccgcggagaggtgaaggccgtggggcctggggaagggctccctgccgcgccccgagacttctagggcgagtttgaaggtgtaggctcggcagtccctcctctcccggcgcgggcggcagcgaggctgggcagagggcagcgcagcgggcagactaggggcatgtctttcccccgcggctgcgtagcgccccgatacttgaaggcggggggcaatccctgttcacaccgcgcttcctcccgccagctggggctgctgcccctcctcagccagctctcgggggaggtggggcgcgaggaggagaggacggcagcctcgcagcctggcggcaacagctcccgcttgggccgggcgagcaacaagcaccggagctggagggacgggattgtagatccggctccgggctcccgggcgggagcgcagcccgtggcatttaaagagacaggc

SEQ ID NO: 15702 - RNA, 3693 nt, Homo sapiens
  source 1..3693: mol_type = other RNA
gctgggattacaggcatgagccactgtgcccggcctaccttctattttcactactgtgttaagcatgaaagaaaatccaactgggttagatacagcaggttctcctaaatgtcttaacccatgtttatcttgttctgctattccatgagcaaagagaataaacacaaagctgtgagagtattaaatatggacactagatttacatttccaacaagaaattcatctccctccaaagtcccagaccagggctagaatgtggttcatttttaacaatcaaagtggcaagatctgtttggtgatcactgtaaaaacaggaaacatagctaatgccctttcatgttgaggtgctacaaaggtccaagcttttaaagactatggcctcaacgtccatgtgtgaaacaagtgtattagaaaattctttaagtcttgttgccttaacttagagatctccaggcaacaggcctgacgatagccatggctgtaccacttaactatgattctattccaactgttcagaatcatatcacaaaatgacttgtacacagtagtttacaacgactcccaagagaggaaaaaaaaaaaaagacgcctcaaaattcactcaacttttgagacagcaatggcaataggcagcagagaagctatgctgcaactgagggcacatatcattgaagatgtcacaggagtttaagagacaggctggaaaaaatctcatactaagcaaacagtagtatctcataccaagcaaaaccaagtagtatctgctcagcctgccgctaacagatctcacaatcaccaactgtgctttaggactgtcaccaaagtcagattcggtgctaaccaggtggcatctatgatcaacgtcgcccctcttatttaacaaagggctctgaaggaggtgttctccaagcaacaaggagactgcttcagtacaagactttgcaccttgaattcaattgcatcaagtgtggatagcaaaataagtatcttaccattgaaatatgtgttcagcctaagattttacccaccagcagaacaaaagtgagggtgagagggatgggccagtgaggggatgggggagaaaaaaaaatcacaggattaccaccaaagccttgttttaaaagggctcccttcactattcaggaagggaagtggaaggagaaattaaccaattcctgccacagcagccctttttggctgcttccacaatagatactttatggagtggcacagccaaccctatctgtgacctgccctgcggataaacacagccaagcaggtttaattagatcaaagacacaaagggctattccctcctttcataacaacgcagctgtaagtgcctacaacagcaggggagaaacaaaggcagcagaacagaaccttaattgaaaccttcccctggctggcccttgacaatgatttacttgtaacctaggaaggggcgggtggagcaggaggtagcaggagcctcagctaagagccagctccagaaggctaattacttgggggttgtggaggagggaggtagcaaagtctttgtttgtagcccgagtttgcttaactatttgttacacttaataggaggctgctgtggttttggtctgctgctcccggaccttgtcatggattcaccagccctgcgctccaggaatcccataaaataaatcaccccagcctcctggatcccatacacagctcagctccgccaaagcagacaagcagctttcgtgctggtcccgcagtggcgactccacaaacccactctggcctttctaccaggattcttccaagcccaggataggaagcaacggcaggaatgggtactccgaactttcccccaaccccacgtgcttaagaatggccgattataaacccagatctaccaaggtttaagtgccaggcaagtccacagtttgctccaccgcggagaggaagacagacagggggccagagggagacgccccccacccccaactaaagtgtttcctacctgctccctctgtccccttcctcctcccccgtccacagccggctgcgcatttcaccaactcttttccaaagggcccaggaatcccagatggggcccagacagtggcaaaagagggaggaagagagggagaaagggagcagcggctgctactgcaaacagttccccttcgcagctctgcgctcagctcgcccatcagtgtgccactgcctctccgtcctcctcctcggagctgggcgcaggggggcgcccgggaggcggcgtagtccgcgccacgttgctgtcgccctcctccggctccgccgggtgcaggtgcgtggcgagctcctgcagcacggccgcgcgcccgatctggtcgttgcgtcgcttctccatgatcaggtcctctagactctggaactcgagcgtgtggctgcgctgcgccgacagctgaatctgcagccggtagggctgcttgccgatgcgcagctcgccgccgatcttgaactcgcgcttgccgtagcggcaccaggcggcgaaactctccgagttgcgccagctcagctcgcgctccttggcacccacgtgcgccagcgcgttgcgcaccacggcgctggagcttagcggcttgtagcggtacagatcgttgaccacgcggccgcgacggccctggctggcgtcagtcaggaagctgttaatcacctccagccggtgcaggtgcaccacctggaagttacccacatatacggcccagtgcgggtactgagcctgcgacacgaactccaccagatcgcccggcttgcacttgttgagcaggttctcgggcgtgtaggtactcagcgccgccgagcccggcgcgaagctcttctggtagatgcattcgtcccggtagaacacggagcattccacctcgtgcagccgcggatcgtagggctgcggctggggcggcggcggcccgtccccaccgtcgggcaagccgccgccatctggcccctgaggcggcggctgcggctccacgtcctcatcgtcattggagaaaatgtaggagaccccaatgcggggcccgtcgtcccggtccacgccagtcgggtcggccgtgggaacttccttgtaacttaggtgggtcaatttctccacctggttgcccatcacgctgcggacacacgttcacaccgccgcaaggggagaaagcgaaaccaactccagggtcatttgcacaggtccccggacaggggctgaggctacctgcacaaactcacccgcggagaggtgaaggccgtggggcctggggaagggctccctgccgcgccccgagacttctagggcgagtttgaaggtgtaggctcggcagtccctcctctcccggcgcgggcggcagcgaggctgggcagagggcagcgcagcgggcagactaggggcatgtctttcccccgcggctgcgtagcgccccgatacttgaaggcggggggcaatccctgttcacaccgcgcttcctcccgccagctggggctgctgcccctcctcagccagctctcgggggaggtggggcgcgaggaggagaggacggcagcctcgcagcctggcggcaacagctcccgcttgggccgggcgagcaacaagcaccggagctggagggacgggattgtagatccggctccgggctcccgggcgggagcgcagcccgtggcatttaaagagacaggcgctcactccccgagctcggg

SEQ ID NO: 15703 - RNA, 3518 nt, Homo sapiens
  source 1..3518: mol_type = other RNA
gctgggattacaggcatgagccactgtgcccggcctaccttctattttcactactgtgttaagcatgaaagaaaatccaactgggttagatacagcaggttctcctaaatgtcttaacccatgtttatcttgttctgctattccatgagcaaagagaataaacacaaagctgtgagagtattaaatatggacactagatttacatttccaacaagaaattcatctccctccaaagtcccagaccagggctagaatgtggttcatttttaacaatcaaagtggcaagatctgtttggtgatcactgtaaaaacaggaaacatagctaatgccctttcatgttgaggtgctacaaaggtccaagcttttaaagactatggcctcaacgtccatgtgtgaaacaagtgtattagaaaattctttaagtcttgttgccttaacttagagatctccaggcaacaggcctgacgatagccatggctgtaccacttaactatgattctattccaactgttcagaatcatatcacaaaatgacttgtacacagtagtttacaacgactcccaagagaggaaaaaaaaaaaaagacgcctcaaaattcactcaacttttgagacagcaatggcaataggcagcagagaagctatgctgcaactgagggcacatatcattgaagatgtcacaggagtttaagagacaggctggaaaaaatctcatactaagcaaacagtagtatctcataccaagcaaaaccaagtagtatctgctcagcctgccgctaacagatctcacaatcaccaactgtgctttaggactgtcaccaaagtcagattcggtgctaaccaggtggcatctatgatcaacgtcgcccctcttatttaacaaagggctctgaaggaggtgttctccaagcaacaaggagactgcttcagtacaagactttgcaccttgaattcaattgcatcaagtgtggatagcaaaataagtatcttaccattgaaatatgtgttcagcctaagattttacccaccagcagaacaaaagtgagggtgagagggatgggccagtgaggggatgggggagaaaaaaaaatcacaggattaccaccaaagccttgttttaaaagggctcccttcactattcaggaagggaagtggaaggagaaattaaccaattcctgccacagcagccctttttggctgcttccacaatagatactttatggagtggcacagccaaccctatctgtgacctgccctgcggataaacacagccaagcaggtttaattagatcaaagacacaaagggctattccctcctttcataacaacgcagctgtaagtgcctacaacagcaggggagaaacaaaggcagcagaacagaaccttaattgaaaccttcccctggctggcccttgacaatgatttacttgtaacctaggaaggggcgggtggagcaggaggtagcaggagcctcagctaagagccagctccagaaggctaattacttgggggttgtggaggagggaggtagcaaagtctttgtttgtagcccgagtttgcttaactatttgttacacttaataggaggctgctgtggttttggtctgctgctcccggaccttgtcatggattcaccagccctgcgctccaggaatcccataaaataaatcaccccagcctcctggatcccatacacagctcagctccgccaaagcagacaagcagctttcgtgctggtcccgcagtggcgactccacaaacccactctggcctttctaccaggattcttccaagcccaggataggaagcaacggcaggaatgggtactccgaactttcccccaaccccacgtgcttaagaatggccgattataaacccagatctaccaaggtttaagtgccaggcaagtccacagtttgctccaccgcggagaggaagacagacagggggccagagggagacgccccccacccccaactaaagtgtttcctacctgctccctctgtccccttcctcctcccccgtccacagccggctgcgcatttcaccaactcttttccaaagggcccaggaatcccagatggggcccagacagtggcaaaagagggaggaagagagggagaaagggagcagcggctgctactgcaaacagttccccttcgcagctctgcgctcagctcgcccatcagtgtgccactgcctctccgtcctcctcctcggagctgggcgcaggggggcgcccgggaggcggcgtagtccgcgccacgttgctgtcgccctcctccggctccgccgggtgcaggtgcgtggcgagctcctgcagcacggccgcgcgcccgatctggtcgttgcgtcgcttctccatgatcaggtcctctagactctggaactcgagcgtgtggctgcgctgcgccgacagctgaatctgcagccggtagggctgcttgccgatgcgcagctcgccgccgatcttgaactcgcgcttgccgtagcggcaccaggcggcgaaactctccgagttgcgccagctcagctcgcgctccttggcacccacgtgcgccagcgcgttgcgcaccacggcgctggagcttagcggcttgtagcggtacagatcgttgaccacgcggccgcgacggccctggctggcgtcagtcaggaagctgttaatcacctccagccggtgcaggtgcaccacctggaagttacccacatatacggcccagtgcgggtactgagcctgcgacacgaactccaccagatcgcccggcttgcacttgttgagcaggttctcgggcgtgtaggtactcagcgccgccgagcccggcgcgaagctcttctggtagatgcattcgtcccggtagaacacggagcattccacctcgtgcagccgcggatcgtagggctgcggctggggcggcggctgcggctccacgtcctcatcgtcattggagaaaatgtaggagaccccaatgcggggcccgtcgtcccggtccacgccagtcgggtcggccgtgggaacttccttgtaacttaggtgggtcaatttctccacctggttgcccatcacgctgcggacacacgttcacaccgccgcaaggggagaaagcgaaaccaactccagggtcatttgcacaggtccccggacaggggctgaggctacccgcggagaggtgaaggccgtggggcctggggaagggctccctgccgcgccccgagacttctagggcgagtttgaaggtgtaggctcggcagtccctcctctcccggcgcgggcggcagcgaggctgggcagagggcagcgcagcgggcagactaggggcatgtctttcccccgcggctgcgtagcgccccgatacttgaaggcggggggcaatccctgttcacaccgcgcttcctcccgccagctggggctgctgcccctcctcagccagctctcgggggaggtggggcgcgaggaggagaggacggcagcctcgcagcctggcggcaacagctcccgcttgggccgggcgagcaac

SEQ ID NO: 15704 - RNA, 5041 nt, Homo sapiens
  source 1..5041: mol_type = other RNA
gctgggattacaggcatgagccactgtgcccggcctagagttgctttttaaggggaaaaaaaccacaggtccttatgaaatattttgaatatagagaaagcacttacttatataaatcccatagaatgaagtcttttctatacaagtaagtgtgttggcacttttaccaaagtctgcctttaataaaatttctcatattatgaataatacaggagctaaatctaagcttaattttagttaacactgcctccatgaaataaaaaccctctcaaattaaaaatctgaactttcttttcaaagtatgtatttctctcacttttcatgcagaggaaggctatttgttgtgtttacctctttctcatctttgaggatttagatttactaagatctgttagatgatgctgaaaaacaatgaacatatttgaaaggaagtgtgttctgattattgcaagaaaagcctgcatttgactgatctcaccaagaaaattcagtttaaagcctttctttggtgatattttagcaattaatcaaggttattgcctaactatataaaattaaattgcaatctaaaaatttccaacctccaaactgttaaaaccgtctctccaacatggttattaatttactgtaaaatgtctttggtgatatctatattcttatgaaaatcttccaaaaaaattaacttacaagagcctatttagatatgaaaccattcataagagacaggtacagataactcaaactttatgcagtaaatttaaaacagaaatgcactttagtaatgaggcactttctcttaaatatttcagtaaagctaaacagttcacaatattatataacacactttttttccttaaataatcagtttaaatttagattacatttgagtgtgtaatgtagttgagcaaagtcattacgtttataaaatgtggcacattactatgggatagatgtttaatgtataaagaaataatatactcctctaagagtagttaaaaggcattacccaagttacctgtactccagactgagtattacctcatcaatgagcattttagtttattttttcatactttgtaaagctgttttgctaatctagagaaaaggccatacatattttgatttctctattaactgatgtgattacttcaattaaagtaatgtttataaaccacagtcattctttatatctaagttcccttgacccttttatacttataatttctaaggcagataaaagagataacaaaatcttttatggaagtaaaggtctttcagtttattgcttaagaaacaacagattaaagaaaacttttagttttagtctctgatgttacagattcagatgattcctataggttatttaaagaattcattttatcattttataagcaccctaaatttataaagctaaccacaaaagttgcctgtacattttttctatacctagtttcttgcaaattctacaatctgacttaagggataattaacggggaatacagtgtattactagacatgaaagtagtcctatccttagaaagctgtagttgaatataccaaaataagtcagttgaagaaatctgtgattctagtagtaataccatatcacttaggaccatcaaaaaaatgtgtacctttctccaaacgacaactgatgcctttctttatgtaagcttttcacgtgttttggcacatattccattgcatttcaataaaaatgttaatgcattatcagtaaataaaagaattctatataaaactattctcagtttcataattgcttcctatatatttccttggaaaatagtgaaattacatatgacaaggcaaccagccaaatttaaagagattttgtagataaaattcatttatgaccattaagttttggctggggggccaaaacatcaaagtctcacttgtgatttttaaaatgcactcttaattcattttgagttaattaaaattccatttgcaaaacactattttaatcgctgacctaggtgtgacaaatttataataatttgtaaaagttcttagggatgtctgggaacagtttcacaccatagaaaaataatttctgtagctagatagtaaattcagttttttcagccatttatagttaatgaaaatctgccttttaaattctgcttgtgagccattccaagaacaaaaacaatgtaacaaaacaaagttaaagtattgccataacctttttcaccaaagttggaacaacaacagaaaaatttaatagactttttgactcaaaaaaagatagaaggaacagataattatgaagtttcagccttttacatagtgaaatatattaagatttagctgtactttgtatgtttgctagagttgtacaatatcttatttctaagaatcattttgaaattcagaaggcattgatttctgatacattttactggaaaatgtgacacatttaccacatatgcagtataaaaactaaatgtgtgtaacacacagattgtgctcgtcatatttctcaaatatttttcctaactttcaagattttttcctaagtttcaaaggttagcttgtttgtttcaaagcaatttccaagtaaggtttttgaaaactgtaaatattaaaagatttaaaatgacagttttcatataatttaaggtaacaagactttctttgacttgcagactaatcctaaaacgaatggaagacttaacaaaactgcaaaatacaggacattttgtatttctgatcttaatgaactcatgtataaaataataatcttctcatttccccaattactacaggatttaaaataaaatacccttaacctattaattttggttagcatagttctatactgcatttattctattttatgcacatagtttggaaatgtgaaaggtaactaacagttttaatctacaactgttttgagacttttgaaatccataaaatagctaatgttatgtgctctaaaaatcctaatatttaaaatcgtcataaccctctgcatgccacaatgacatatacctaaggccaacttaaaaagagaaataatgcactcattaaataacagcaacaatgtaatgatacatgaaatgggctatacaatgacgtttcatgaagcagcacctgcttgtcataaggcattatgaaagaagattaaccttacttacacattacttttatcagaagtaaatgtgatcagctgccaacattttgaatggttgggaatctaacttcagttcaagaggtcacatacattttcaatctggagggctaacatgccttccttgtgcaattggtagactacacggacagatgcttagaatgtctacaattatattgtgctctaatgttacagaataattggaattcttggcaaaaggacttgcacactcaagaatgaactttttttcacacaaaaagcttatcaagaacaagacagtggctcaaaaaccacttttctaaatatacttccatacaaaataatttcaagatataattattagtttcttgtagagtacgctatttaaacaagaataaaagagtaagtatgtgaaaactgcaacaccacaaaaattgagccattttactagtgtaattaaacattagaacaatcttggaacaggcaagcaaaatattcagaagggtgaatcatggcggcacagctaactgatttttaccatgacttgcacactttgagacaacacaaataccttatgcagatggttcagtagcagaatggcacttggtttgctcctaatagaaacaacatgaatgcaactgacaatttagagatagacaatggccttatttgcatgctgaaaatctggttgtgttcctctagtccacacaccgttaactgtgcaatctgttgacgagtaaacaaatagtgcaggattcatctcagtgaggtctgggccccttggtctaaccgaaatcaattcttggtcgatactgcagtaccatagggtatgactgatacaaagggccatcctgagagcagacttgcgaagctgagcagttcagacaccgaaagttttcgcctcttagtcgccatcttgtcatgtagatgaattccatagtatgatccttccccataatttcaccattgcacagcacatccaactcataagaacttggaagttttagttttaaacttagaaattttttaatagttcccacagttacacgtgtagaacatcgaatgaatttcttcattaaaccctttactacattgtcccctgattgcccattatttcgtaaacaatctagacagatagcaatttgtgggtcacttctgtgataatctttatcatcttcattttcatcaccttcttcatctactttcggtttgtcagcttttgaagtatcatcttgtccattttcttgaggcttatttttcttccaaaattcagattcacgctcaagttcttgttctcgtagtccagggaccagcttaaatataatttcctctaatgtattgtccaacatgtatggaggcattccgtcactgttgttggcttgatcagataccctttacagatatagcaggtaatgtaaggattaaaatctttcaccaagtgtttcctttgggtagccattcgtggctagtgaagactggctttagtagtctgggcaaagaggggtcctaagtagatgaaagtctgatcccaggagctggtgtgtcgttcccagtaggatgtcctgaggcatgagaactagcatccagatttatcatgagatcgttgatcatcactccttttggtggttccgctttcccatgtccagcggccgccaccgccgccgctcctcgcccgccagcgcgccggcctcagagtgaaggaaagtgaaacagaaacagcacccgccgcggcctggccggtccccgcgccccgtctgctctccccctgcaggcgggagcgcgccggctctgtggggccactcggctcaggcccgacagggcgcggcgggcctcggggcccaggtccggtgccgcctccaagggcaactccacccacttccaaccggcggcaccgcccgccccgcc

SEQ ID NO: 15705 - RNA, 5110 nt, Homo sapiens
  source 1..5110: mol_type = other RNA
gctgggattacaggcatgagccactgtgcccggcctagagttgctttttaaggggaaaaaaaccacaggtccttatgaaatattttgaatatagagaaagcacttacttatataaatcccatagaatgaagtcttttctatacaagtaagtgtgttggcacttttaccaaagtctgcctttaataaaatttctcatattatgaataatacaggagctaaatctaagcttaattttagttaacactgcctccatgaaataaaaaccctctcaaattaaaaatctgaactttcttttcaaagtatgtatttctctcacttttcatgcagaggaaggctatttgttgtgtttacctctttctcatctttgaggatttagatttactaagatctgttagatgatgctgaaaaacaatgaacatatttgaaaggaagtgtgttctgattattgcaagaaaagcctgcatttgactgatctcaccaagaaaattcagtttaaagcctttctttggtgatattttagcaattaatcaaggttattgcctaactatataaaattaaattgcaatctaaaaatttccaacctccaaactgttaaaaccgtctctccaacatggttattaatttactgtaaaatgtctttggtgatatctatattcttatgaaaatcttccaaaaaaattaacttacaagagcctatttagatatgaaaccattcataagagacaggtacagataactcaaactttatgcagtaaatttaaaacagaaatgcactttagtaatgaggcactttctcttaaatatttcagtaaagctaaacagttcacaatattatataacacactttttttccttaaataatcagtttaaatttagattacatttgagtgtgtaatgtagttgagcaaagtcattacgtttataaaatgtggcacattactatgggatagatgtttaatgtataaagaaataatatactcctctaagagtagttaaaaggcattacccaagttacctgtactccagactgagtattacctcatcaatgagcattttagtttattttttcatactttgtaaagctgttttgctaatctagagaaaaggccatacatattttgatttctctattaactgatgtgattacttcaattaaagtaatgtttataaaccacagtcattctttatatctaagttcccttgacccttttatacttataatttctaaggcagataaaagagataacaaaatcttttatggaagtaaaggtctttcagtttattgcttaagaaacaacagattaaagaaaacttttagttttagtctctgatgttacagattcagatgattcctataggttatttaaagaattcattttatcattttataagcaccctaaatttataaagctaaccacaaaagttgcctgtacattttttctatacctagtttcttgcaaattctacaatctgacttaagggataattaacggggaatacagtgtattactagacatgaaagtagtcctatccttagaaagctgtagttgaatataccaaaataagtcagttgaagaaatctgtgattctagtagtaataccatatcacttaggaccatcaaaaaaatgtgtacctttctccaaacgacaactgatgcctttctttatgtaagcttttcacgtgttttggcacatattccattgcatttcaataaaaatgttaatgcattatcagtaaataaaagaattctatataaaactattctcagtttcataattgcttcctatatatttccttggaaaatagtgaaattacatatgacaaggcaaccagccaaatttaaagagattttgtagataaaattcatttatgaccattaagttttggctggggggccaaaacatcaaagtctcacttgtgatttttaaaatgcactcttaattcattttgagttaattaaaattccatttgcaaaacactattttaatcgctgacctaggtgtgacaaatttataataatttgtaaaagttcttagggatgtctgggaacagtttcacaccatagaaaaataatttctgtagctagatagtaaattcagttttttcagccatttatagttaatgaaaatctgccttttaaattctgcttgtgagccattccaagaacaaaaacaatgtaacaaaacaaagttaaagtattgccataacctttttcaccaaagttggaacaacaacagaaaaatttaatagactttttgactcaaaaaaagatagaaggaacagataattatgaagtttcagccttttacatagtgaaatatattaagatttagctgtactttgtatgtttgctagagttgtacaatatcttatttctaagaatcattttgaaattcagaaggcattgatttctgatacattttactggaaaatgtgacacatttaccacatatgcagtataaaaactaaatgtgtgtaacacacagattgtgctcgtcatatttctcaaatatttttcctaactttcaagattttttcctaagtttcaaaggttagcttgtttgtttcaaagcaatttccaagtaaggtttttgaaaactgtaaatattaaaagatttaaaatgacagttttcatataatttaaggtaacaagactttctttgacttgcagactaatcctaaaacgaatggaagacttaacaaaactgcaaaatacaggacattttgtatttctgatcttaatgaactcatgtataaaataataatcttctcatttccccaattactacaggatttaaaataaaatacccttaacctattaattttggttagcatagttctatactgcatttattctattttatgcacatagtttggaaatgtgaaaggtaactaacagttttaatctacaactgttttgagacttttgaaatccataaaatagctaatgttatgtgctctaaaaatcctaatatttaaaatcgtcataaccctctgcatgccacaatgacatatacctaaggccaacttaaaaagagaaataatgcactcattaaataacagcaacaatgtaatgatacatgaaatgggctatacaatgacgtttcatgaagcagcacctgcttgtcataaggcattatgaaagaagattaaccttacttacacattacttttatcagaagtaaatgtgatcagctgccaacattttgaatggttgggaatctaacttcagttcaagaggtcacatacattttcaatctggagggctaacatgccttccttgtgcaattggtagactacacggacagatgcttagaatgtctacaattatattgtgctctaatgttacagaataattggaattcttggcaaaaggacttgcacactcaagaatgaactttttttcacacaaaaagcttatcaagaacaagacagtggctcaaaaaccacttttctaaatatacttccatacaaaataatttcaagatataattattagtttcttgtagagtacgctatttaaacaagaataaaagagtaagtatgtgaaaactgcaacaccacaaaaattgagccattttactagtgtaattaaacattagaacaatcttggaacaggcaagcaaaatattcagaagggtgaatcatggcggcacagctaactgatttttaccatgacttgcacactttgagacaacacaaataccttatgcagatggttcagtagcagaatggcacttggtttgctcctaatagaaacaacatgaatgcaactgacaatttagagatagacaatggccttatttgcatgctgaaaatctggttgtgttcctctagtccacacaccgttaactgtgcaatctgttgacgagtaaacaaatagtgcaggattcatctcagtgaggtctgggccccttggtctaaccgaaatcaattcttggtcgatactgcagtaccatagggtatgactgatacaaagggccatcctgagagcagacttgcgaagctgagcagttcagacaccgaaagttttcgcctcttagtcgccatcttgtcatgtagatgaattccatagtatgatccttccccataatttcaccattgcacagcacatccaactcataagaacttggaagttttagttttaaacttagaaattttttaatagttcccacagttacacgtgtagaacatcgaatgaatttcttcattaaaccctttactacattgtcccctgattgcccattatttcgtaaacaatctagacagatagcaatttgtgggtcacttctgtgataatctttatcatcttcattttcatcaccttcttcatctactttcggtttgtcagcttttgaagtatcatcttgtccattttcttgaggcttatttttcttccaaaattcagattcacgctcaagttcttgttctcgtagtccagggaccagcttaaatataatttcctctaatgtattgtccaacctcaacatttctaatggatttgtctcatgaacttggttgccacaccttgggcaatcattgctatcttcaaagtgctgaacaatacaagtcttacagaatgtatggaggcattccgtcactgttgttggcttgatcagataccctttacagatatagcaggtaatgtaaggattaaaatctttcaccaagtgtttcctttgggtagccattcgtggctagtgaagactggctttagtagtctgggcaaagaggggtcctaagtagatgaaagtctgatcccaggagctggtgtgtcgttcccagtaggatgtcctgaggcatgagaactagcatccagatttatcatgagatcgttgatcatcactccttttggtggttccgctttcccatgtccactgcgaatgtgcagggaataggctctacgtgtaatcatcctatcctcttgggaaaccgtattcgtgcgtgtaacagaaagcaagcataattaaaagacagggaatcagggttctggcccttacccctgtatgaccttcagcaaaccgtttcatatctgagcctgggtctcggcttcctcctctataagttgggattaactgccttgcctttcccacaggtttgccatgaaac

SEQ ID NO: 15706 - RNA, 5049 nt, Homo sapiens
  source 1..5049: mol_type = other RNA
gctgggattacaggcatgagccactgtgcccggcctagagttgctttttaaggggaaaaaaaccacaggtccttatgaaatattttgaatatagagaaagcacttacttatataaatcccatagaatgaagtcttttctatacaagtaagtgtgttggcacttttaccaaagtctgcctttaataaaatttctcatattatgaataatacaggagctaaatctaagcttaattttagttaacactgcctccatgaaataaaaaccctctcaaattaaaaatctgaactttcttttcaaagtatgtatttctctcacttttcatgcagaggaaggctatttgttgtgtttacctctttctcatctttgaggatttagatttactaagatctgttagatgatgctgaaaaacaatgaacatatttgaaaggaagtgtgttctgattattgcaagaaaagcctgcatttgactgatctcaccaagaaaattcagtttaaagcctttctttggtgatattttagcaattaatcaaggttattgcctaactatataaaattaaattgcaatctaaaaatttccaacctccaaactgttaaaaccgtctctccaacatggttattaatttactgtaaaatgtctttggtgatatctatattcttatgaaaatcttccaaaaaaattaacttacaagagcctatttagatatgaaaccattcataagagacaggtacagataactcaaactttatgcagtaaatttaaaacagaaatgcactttagtaatgaggcactttctcttaaatatttcagtaaagctaaacagttcacaatattatataacacactttttttccttaaataatcagtttaaatttagattacatttgagtgtgtaatgtagttgagcaaagtcattacgtttataaaatgtggcacattactatgggatagatgtttaatgtataaagaaataatatactcctctaagagtagttaaaaggcattacccaagttacctgtactccagactgagtattacctcatcaatgagcattttagtttattttttcatactttgtaaagctgttttgctaatctagagaaaaggccatacatattttgatttctctattaactgatgtgattacttcaattaaagtaatgtttataaaccacagtcattctttatatctaagttcccttgacccttttatacttataatttctaaggcagataaaagagataacaaaatcttttatggaagtaaaggtctttcagtttattgcttaagaaacaacagattaaagaaaacttttagttttagtctctgatgttacagattcagatgattcctataggttatttaaagaattcattttatcattttataagcaccctaaatttataaagctaaccacaaaagttgcctgtacattttttctatacctagtttcttgcaaattctacaatctgacttaagggataattaacggggaatacagtgtattactagacatgaaagtagtcctatccttagaaagctgtagttgaatataccaaaataagtcagttgaagaaatctgtgattctagtagtaataccatatcacttaggaccatcaaaaaaatgtgtacctttctccaaacgacaactgatgcctttctttatgtaagcttttcacgtgttttggcacatattccattgcatttcaataaaaatgttaatgcattatcagtaaataaaagaattctatataaaactattctcagtttcataattgcttcctatatatttccttggaaaatagtgaaattacatatgacaaggcaaccagccaaatttaaagagattttgtagataaaattcatttatgaccattaagttttggctggggggccaaaacatcaaagtctcacttgtgatttttaaaatgcactcttaattcattttgagttaattaaaattccatttgcaaaacactattttaatcgctgacctaggtgtgacaaatttataataatttgtaaaagttcttagggatgtctgggaacagtttcacaccatagaaaaataatttctgtagctagatagtaaattcagttttttcagccatttatagttaatgaaaatctgccttttaaattctgcttgtgagccattccaagaacaaaaacaatgtaacaaaacaaagttaaagtattgccataacctttttcaccaaagttggaacaacaacagaaaaatttaatagactttttgactcaaaaaaagatagaaggaacagataattatgaagtttcagccttttacatagtgaaatatattaagatttagctgtactttgtatgtttgctagagttgtacaatatcttatttctaagaatcattttgaaattcagaaggcattgatttctgatacattttactggaaaatgtgacacatttaccacatatgcagtataaaaactaaatgtgtgtaacacacagattgtgctcgtcatatttctcaaatatttttcctaactttcaagattttttcctaagtttcaaaggttagcttgtttgtttcaaagcaatttccaagtaaggtttttgaaaactgtaaatattaaaagatttaaaatgacagttttcatataatttaaggtaacaagactttctttgacttgcagactaatcctaaaacgaatggaagacttaacaaaactgcaaaatacaggacattttgtatttctgatcttaatgaactcatgtataaaataataatcttctcatttccccaattactacaggatttaaaataaaatacccttaacctattaattttggttagcatagttctatactgcatttattctattttatgcacatagtttggaaatgtgaaaggtaactaacagttttaatctacaactgttttgagacttttgaaatccataaaatagctaatgttatgtgctctaaaaatcctaatatttaaaatcgtcataaccctctgcatgccacaatgacatatacctaaggccaacttaaaaagagaaataatgcactcattaaataacagcaacaatgtaatgatacatgaaatgggctatacaatgacgtttcatgaagcagcacctgcttgtcataaggcattatgaaagaagattaaccttacttacacattacttttatcagaagtaaatgtgatcagctgccaacattttgaatggttgggaatctaacttcagttcaagaggtcacatacattttcaatctggagggctaacatgccttccttgtgcaattggtagactacacggacagatgcttagaatgtctacaattatattgtgctctaatgttacagaataattggaattcttggcaaaaggacttgcacactcaagaatgaactttttttcacacaaaaagcttatcaagaacaagacagtggctcaaaaaccacttttctaaatatacttccatacaaaataatttcaagatataattattagtttcttgtagagtacgctatttaaacaagaataaaagagtaagtatgtgaaaactgcaacaccacaaaaattgagccattttactagtgtaattaaacattagaacaatcttggaacaggcaagcaaaatattcagaagggtgaatcatggcggcacagctaactgatttttaccatgacttgcacactttgagacaacacaaataccttatgcagatggttcagtagcagaatggcacttggtttgctcctaatagaaacaacatgaatgcaactgacaatttagagatagacaatggccttatttgcatgctgaaaatctggttgtgttcctctagtccacacaccgttaactgtgcaatctgttgacgagtaaacaaatagtgcaggattcatctcagtgaggtctgggccccttggtctaaccgaaatcaattcttggtcgatactgcagtaccatagggtatgactgatacaaagggccatcctgagagcagacttgcgaagctgagcagttcagacaccgaaagttttcgcctcttagtcgccatcttgtcatgtagatgaattccatagtatgatccttccccataatttcaccattgcacagcacatccaactcataagaacttggaagttttagttttaaacttagaaattttttaatagttcccacagttacacgtgtagaacatcgaatgaatttcttcattaaaccctttactacattgtcccctgattgcccattatttcgtaaacaatctagacagatagcaatttgtgggtcacttctgtgataatctttatcatcttcattttcatcaccttcttcatctactttcggtttgtcagcttttgaagtatcatcttgtccattttcttgaggcttatttttcttccaaaattcagattcacgctcaagttcttgttctcgtagtccagggaccagcttaaatataatttcctctaatgtattgtccaacctcaacatttctaatggatttgtctcatgaacttggttgccacaccttgggcaatcattgctatcttcaaagtgctgaacaatacaagtcttacagaatgtatggaggcattccgtcactgttgttggcttgatcagataccctttacagatatagcaggtaatgtaaggattaaaatctttcaccaagtgtttcctttgggtagccattcgtggctagtgaagactggctttagtagtctgggcaaagaggggtcctaagtagatgaaagtctgatcccaggagctggtgtgtcgttcccagtaggatgtcctgaggcatgagaactagcatccagatttatcatgagatcgttgatcatcactccttttggtggttccgctttcccatgtccagcggccgccaccgccgccgctcctcgcccgccagcgcgccggcctcagagtgaaggaaagtgaaacagaaacagcacccgccgcggcctggccggtccccgcgccccgtctgctctccccctgcaggcgggagcgcgccggctctgtggggccactcggctcaggcccgac

SEQ ID NO: 15707 - RNA, 5052 nt, Homo sapiens
  source 1..5052: mol_type = other RNA
gctgggattacaggcatgagccactgtgcccggcctagagttgctttttaaggggaaaaaaaccacaggtccttatgaaatattttgaatatagagaaagcacttacttatataaatcccatagaatgaagtcttttctatacaagtaagtgtgttggcacttttaccaaagtctgcctttaataaaatttctcatattatgaataatacaggagctaaatctaagcttaattttagttaacactgcctccatgaaataaaaaccctctcaaattaaaaatctgaactttcttttcaaagtatgtatttctctcacttttcatgcagaggaaggctatttgttgtgtttacctctttctcatctttgaggatttagatttactaagatctgttagatgatgctgaaaaacaatgaacatatttgaaaggaagtgtgttctgattattgcaagaaaagcctgcatttgactgatctcaccaagaaaattcagtttaaagcctttctttggtgatattttagcaattaatcaaggttattgcctaactatataaaattaaattgcaatctaaaaatttccaacctccaaactgttaaaaccgtctctccaacatggttattaatttactgtaaaatgtctttggtgatatctatattcttatgaaaatcttccaaaaaaattaacttacaagagcctatttagatatgaaaccattcataagagacaggtacagataactcaaactttatgcagtaaatttaaaacagaaatgcactttagtaatgaggcactttctcttaaatatttcagtaaagctaaacagttcacaatattatataacacactttttttccttaaataatcagtttaaatttagattacatttgagtgtgtaatgtagttgagcaaagtcattacgtttataaaatgtggcacattactatgggatagatgtttaatgtataaagaaataatatactcctctaagagtagttaaaaggcattacccaagttacctgtactccagactgagtattacctcatcaatgagcattttagtttattttttcatactttgtaaagctgttttgctaatctagagaaaaggccatacatattttgatttctctattaactgatgtgattacttcaattaaagtaatgtttataaaccacagtcattctttatatctaagttcccttgacccttttatacttataatttctaaggcagataaaagagataacaaaatcttttatggaagtaaaggtctttcagtttattgcttaagaaacaacagattaaagaaaacttttagttttagtctctgatgttacagattcagatgattcctataggttatttaaagaattcattttatcattttataagcaccctaaatttataaagctaaccacaaaagttgcctgtacattttttctatacctagtttcttgcaaattctacaatctgacttaagggataattaacggggaatacagtgtattactagacatgaaagtagtcctatccttagaaagctgtagttgaatataccaaaataagtcagttgaagaaatctgtgattctagtagtaataccatatcacttaggaccatcaaaaaaatgtgtacctttctccaaacgacaactgatgcctttctttatgtaagcttttcacgtgttttggcacatattccattgcatttcaataaaaatgttaatgcattatcagtaaataaaagaattctatataaaactattctcagtttcataattgcttcctatatatttccttggaaaatagtgaaattacatatgacaaggcaaccagccaaatttaaagagattttgtagataaaattcatttatgaccattaagttttggctggggggccaaaacatcaaagtctcacttgtgatttttaaaatgcactcttaattcattttgagttaattaaaattccatttgcaaaacactattttaatcgctgacctaggtgtgacaaatttataataatttgtaaaagttcttagggatgtctgggaacagtttcacaccatagaaaaataatttctgtagctagatagtaaattcagttttttcagccatttatagttaatgaaaatctgccttttaaattctgcttgtgagccattccaagaacaaaaacaatgtaacaaaacaaagttaaagtattgccataacctttttcaccaaagttggaacaacaacagaaaaatttaatagactttttgactcaaaaaaagatagaaggaacagataattatgaagtttcagccttttacatagtgaaatatattaagatttagctgtactttgtatgtttgctagagttgtacaatatcttatttctaagaatcattttgaaattcagaaggcattgatttctgatacattttactggaaaatgtgacacatttaccacatatgcagtataaaaactaaatgtgtgtaacacacagattgtgctcgtcatatttctcaaatatttttcctaactttcaagattttttcctaagtttcaaaggttagcttgtttgtttcaaagcaatttccaagtaaggtttttgaaaactgtaaatattaaaagatttaaaatgacagttttcatataatttaaggtaacaagactttctttgacttgcagactaatcctaaaacgaatggaagacttaacaaaactgcaaaatacaggacattttgtatttctgatcttaatgaactcatgtataaaataataatcttctcatttccccaattactacaggatttaaaataaaatacccttaacctattaattttggttagcatagttctatactgcatttattctattttatgcacatagtttggaaatgtgaaaggtaactaacagttttaatctacaactgttttgagacttttgaaatccataaaatagctaatgttatgtgctctaaaaatcctaatatttaaaatcgtcataaccctctgcatgccacaatgacatatacctaaggccaacttaaaaagagaaataatgcactcattaaataacagcaacaatgtaatgatacatgaaatgggctatacaatgacgtttcatgaagcagcacctgcttgtcataaggcattatgaaagaagattaaccttacttacacattacttttatcagaagtaaatgtgatcagctgccaacattttgaatggttgggaatctaacttcagttcaagaggtcacatacattttcaatctggagggctaacatgccttccttgtgcaattggtagactacacggacagatgcttagaatgtctacaattatattgtgctctaatgttacagaataattggaattcttggcaaaaggacttgcacactcaagaatgaactttttttcacacaaaaagcttatcaagaacaagacagtggctcaaaaaccacttttctaaatatacttccatacaaaataatttcaagatataattattagtttcttgtagagtacgctatttaaacaagaataaaagagtaagtatgtgaaaactgcaacaccacaaaaattgagccattttactagtgtaattaaacattagaacaatcttggaacaggcaagcaaaatattcagaagggtgaatcatggcggcacagctaactgatttttaccatgacttgcacactttgagacaacacaaataccttatgcagatggttcagtagcagaatggcacttggtttgctcctaatagaaacaacatgaatgcaactgacaatttagagatagacaatggccttatttgcatgctgaaaatctggttgtgttcctctagtccacacaccgttaactgtgcaatctgttgacgagtaaacaaatagtgcaggattcatctcagtgaggtctgggccccttggtctaaccgaaatcaattcttggtcgatactgcagtaccatagggtatgactgatacaaagggccatcctgagagcagacttgcgaagctgagcagttcagacaccgaaagttttcgcctcttagtcgccatcttgtcatgtagatgaattccatagtatgatccttccccataatttcaccattgcacagcacatccaactcataagaacttggaagttttagttttaaacttagaaattttttaatagttcccacagttacacgtgtagaacatcgaatgaatttcttcattaaaccctttactacattgtcccctgattgcccattatttcgtaaacaatctagacagatagcaatttgtgggtcacttctgtgataatctttatcatcttcattttcatcaccttcttcatctactttcggtttgtcagcttttgaagtatcatcttgtccattttcttgaggcttatttttcttccaaaattcagattcacgctcaagttcttgttctcgtagtccagggaccagcttaaatataatttcctctaatgtattgtccaacctcaacatttctaatggatttgtctcatgaacttggttgccacaccttgggcaatcattgctatcttcaaagtgctgaacaatacaagtcttacagaatgtatggaggcattccgtcactgttgttggcttgatcagataccctttacagatatagcaggtaatgtaaggattaaaatctttcaccaagtgtttcctttgggtagccattcgtggctagtgaagactggctttagtagtctgggcaaagaggggtcctaagtagatgaaagtctgatcccaggagctggtgtgtcgttcccagtaggatgtcctgaggcatgagaactagcatccagatttatcatgagatcgttgatcatcactccttttggtggttccgctttcccatgtcctgagaatttgtctcttcagctgcgtcttccccaagtctgtcccacctgcgccgaagtggggacaaagccatcccttgatttgcaccttatctgaaaatgactgacaaacttgttactgtagtgtgggtccagagatcatggtcgttgacaactataagcaaacgggaacgttgtg

SEQ ID NO: 15708 - RNA, 5058 nt, Homo sapiens
  source 1..5058: mol_type = other RNA
gctgggattacaggcatgagccactgtgcccggcctagagttgctttttaaggggaaaaaaaccacaggtccttatgaaatattttgaatatagagaaagcacttacttatataaatcccatagaatgaagtcttttctatacaagtaagtgtgttggcacttttaccaaagtctgcctttaataaaatttctcatattatgaataatacaggagctaaatctaagcttaattttagttaacactgcctccatgaaataaaaaccctctcaaattaaaaatctgaactttcttttcaaagtatgtatttctctcacttttcatgcagaggaaggctatttgttgtgtttacctctttctcatctttgaggatttagatttactaagatctgttagatgatgctgaaaaacaatgaacatatttgaaaggaagtgtgttctgattattgcaagaaaagcctgcatttgactgatctcaccaagaaaattcagtttaaagcctttctttggtgatattttagcaattaatcaaggttattgcctaactatataaaattaaattgcaatctaaaaatttccaacctccaaactgttaaaaccgtctctccaacatggttattaatttactgtaaaatgtctttggtgatatctatattcttatgaaaatcttccaaaaaaattaacttacaagagcctatttagatatgaaaccattcataagagacaggtacagataactcaaactttatgcagtaaatttaaaacagaaatgcactttagtaatgaggcactttctcttaaatatttcagtaaagctaaacagttcacaatattatataacacactttttttccttaaataatcagtttaaatttagattacatttgagtgtgtaatgtagttgagcaaagtcattacgtttataaaatgtggcacattactatgggatagatgtttaatgtataaagaaataatatactcctctaagagtagttaaaaggcattacccaagttacctgtactccagactgagtattacctcatcaatgagcattttagtttattttttcatactttgtaaagctgttttgctaatctagagaaaaggccatacatattttgatttctctattaactgatgtgattacttcaattaaagtaatgtttataaaccacagtcattctttatatctaagttcccttgacccttttatacttataatttctaaggcagataaaagagataacaaaatcttttatggaagtaaaggtctttcagtttattgcttaagaaacaacagattaaagaaaacttttagttttagtctctgatgttacagattcagatgattcctataggttatttaaagaattcattttatcattttataagcaccctaaatttataaagctaaccacaaaagttgcctgtacattttttctatacctagtttcttgcaaattctacaatctgacttaagggataattaacggggaatacagtgtattactagacatgaaagtagtcctatccttagaaagctgtagttgaatataccaaaataagtcagttgaagaaatctgtgattctagtagtaataccatatcacttaggaccatcaaaaaaatgtgtacctttctccaaacgacaactgatgcctttctttatgtaagcttttcacgtgttttggcacatattccattgcatttcaataaaaatgttaatgcattatcagtaaataaaagaattctatataaaactattctcagtttcataattgcttcctatatatttccttggaaaatagtgaaattacatatgacaaggcaaccagccaaatttaaagagattttgtagataaaattcatttatgaccattaagttttggctggggggccaaaacatcaaagtctcacttgtgatttttaaaatgcactcttaattcattttgagttaattaaaattccatttgcaaaacactattttaatcgctgacctaggtgtgacaaatttataataatttgtaaaagttcttagggatgtctgggaacagtttcacaccatagaaaaataatttctgtagctagatagtaaattcagttttttcagccatttatagttaatgaaaatctgccttttaaattctgcttgtgagccattccaagaacaaaaacaatgtaacaaaacaaagttaaagtattgccataacctttttcaccaaagttggaacaacaacagaaaaatttaatagactttttgactcaaaaaaagatagaaggaacagataattatgaagtttcagccttttacatagtgaaatatattaagatttagctgtactttgtatgtttgctagagttgtacaatatcttatttctaagaatcattttgaaattcagaaggcattgatttctgatacattttactggaaaatgtgacacatttaccacatatgcagtataaaaactaaatgtgtgtaacacacagattgtgctcgtcatatttctcaaatatttttcctaactttcaagattttttcctaagtttcaaaggttagcttgtttgtttcaaagcaatttccaagtaaggtttttgaaaactgtaaatattaaaagatttaaaatgacagttttcatataatttaaggtaacaagactttctttgacttgcagactaatcctaaaacgaatggaagacttaacaaaactgcaaaatacaggacattttgtatttctgatcttaatgaactcatgtataaaataataatcttctcatttccccaattactacaggatttaaaataaaatacccttaacctattaattttggttagcatagttctatactgcatttattctattttatgcacatagtttggaaatgtgaaaggtaactaacagttttaatctacaactgttttgagacttttgaaatccataaaatagctaatgttatgtgctctaaaaatcctaatatttaaaatcgtcataaccctctgcatgccacaatgacatatacctaaggccaacttaaaaagagaaataatgcactcattaaataacagcaacaatgtaatgatacatgaaatgggctatacaatgacgtttcatgaagcagcacctgcttgtcataaggcattatgaaagaagattaaccttacttacacattacttttatcagaagtaaatgtgatcagctgccaacattttgaatggttgggaatctaacttcagttcaagaggtcacatacattttcaatctggagggctaacatgccttccttgtgcaattggtagactacacggacagatgcttagaatgtctacaattatattgtgctctaatgttacagaataattggaattcttggcaaaaggacttgcacactcaagaatgaactttttttcacacaaaaagcttatcaagaacaagacagtggctcaaaaaccacttttctaaatatacttccatacaaaataatttcaagatataattattagtttcttgtagagtacgctatttaaacaagaataaaagagtaagtatgtgaaaactgcaacaccacaaaaattgagccattttactagtgtaattaaacattagaacaatcttggaacaggcaagcaaaatattcagaagggtgaatcatggcggcacagctaactgatttttaccatgacttgcacactttgagacaacacaaataccttatgcagatggttcagtagcagaatggcacttggtttgctcctaatagaaacaacatgaatgcaactgacaatttagagatagacaatggccttatttgcatgctgaaaatctggttgtgttcctctagtccacacaccgttaactgtgcaatctgttgacgagtaaacaaatagtgcaggattcatctcagtgaggtctgggccccttggtctaaccgaaatcaattcttggtcgatactgcagtaccatagggtatgactgatacaaagggccatcctgagagcagacttgcgaagctgagcagttcagacaccgaaagttttcgcctcttagtcgccatcttgtcatgtagatgaattccatagtatgatccttccccataatttcaccattgcacagcacatccaactcataagaacttggaagttttagttttaaacttagaaattttttaatagttcccacagttacacgtgtagaacatcgaatgaatttcttcattaaaccctttactacattgtcccctgattgcccattatttcgtaaacaatctagacagatagcaatttgtgggtcacttctgtgataatctttatcatcttcattttcatcaccttcttcatctactttcggtttgtcagcttttgaagtatcatcttgtccattttcttgaggcttatttttcttccaaaattcagattcacgctcaagttcttgttctcgtagtccagggaccagcttaaatataatttcctctaatgtattgtccaacctcaacatttctaatggatttgtctcatgaacttggttgccacaccttgggcaatcattgctatcttcaaagtgctgaacaatacaagtcttacagaatgtatggaggcattccgtcactgttgttggcttgatcagataccctttacagatatagcaggtaatgtaaggattaaaatctttcaccaagtgtttcctttgggtagccattcgtggctagtgaagactggctttagtagtctgggcaaagaggggtcctaagtagatgaaagtctgatcccaggagctggtgtgtcgttcccagtaggatgtcctgaggcatgagaactagcatccagatttatcatgagatcgttgatcatcactccttttggtggttccgctttcccatgtctgtagtggcccgaccttggcaaggagaaattcgaaacttctcaggccggagacttcgaatcgtacagcctctgagggggcaccttctccccccacagacggaggaagcgtgcccttgaatagatggaaggcagctcgaatgtcagtatgcctccctggcgatggtcaagtccaggcttcccg

SEQ ID NO: 15709 - RNA, 4964 nt, Homo sapiens
  source 1..4964: mol_type = other RNA
gctgggattacaggcatgagccactgtgcccggcctagagttgctttttaaggggaaaaaaaccacaggtccttatgaaatattttgaatatagagaaagcacttacttatataaatcccatagaatgaagtcttttctatacaagtaagtgtgttggcacttttaccaaagtctgcctttaataaaatttctcatattatgaataatacaggagctaaatctaagcttaattttagttaacactgcctccatgaaataaaaaccctctcaaattaaaaatctgaactttcttttcaaagtatgtatttctctcacttttcatgcagaggaaggctatttgttgtgtttacctctttctcatctttgaggatttagatttactaagatctgttagatgatgctgaaaaacaatgaacatatttgaaaggaagtgtgttctgattattgcaagaaaagcctgcatttgactgatctcaccaagaaaattcagtttaaagcctttctttggtgatattttagcaattaatcaaggttattgcctaactatataaaattaaattgcaatctaaaaatttccaacctccaaactgttaaaaccgtctctccaacatggttattaatttactgtaaaatgtctttggtgatatctatattcttatgaaaatcttccaaaaaaattaacttacaagagcctatttagatatgaaaccattcataagagacaggtacagataactcaaactttatgcagtaaatttaaaacagaaatgcactttagtaatgaggcactttctcttaaatatttcagtaaagctaaacagttcacaatattatataacacactttttttccttaaataatcagtttaaatttagattacatttgagtgtgtaatgtagttgagcaaagtcattacgtttataaaatgtggcacattactatgggatagatgtttaatgtataaagaaataatatactcctctaagagtagttaaaaggcattacccaagttacctgtactccagactgagtattacctcatcaatgagcattttagtttattttttcatactttgtaaagctgttttgctaatctagagaaaaggccatacatattttgatttctctattaactgatgtgattacttcaattaaagtaatgtttataaaccacagtcattctttatatctaagttcccttgacccttttatacttataatttctaaggcagataaaagagataacaaaatcttttatggaagtaaaggtctttcagtttattgcttaagaaacaacagattaaagaaaacttttagttttagtctctgatgttacagattcagatgattcctataggttatttaaagaattcattttatcattttataagcaccctaaatttataaagctaaccacaaaagttgcctgtacattttttctatacctagtttcttgcaaattctacaatctgacttaagggataattaacggggaatacagtgtattactagacatgaaagtagtcctatccttagaaagctgtagttgaatataccaaaataagtcagttgaagaaatctgtgattctagtagtaataccatatcacttaggaccatcaaaaaaatgtgtacctttctccaaacgacaactgatgcctttctttatgtaagcttttcacgtgttttggcacatattccattgcatttcaataaaaatgttaatgcattatcagtaaataaaagaattctatataaaactattctcagtttcataattgcttcctatatatttccttggaaaatagtgaaattacatatgacaaggcaaccagccaaatttaaagagattttgtagataaaattcatttatgaccattaagttttggctggggggccaaaacatcaaagtctcacttgtgatttttaaaatgcactcttaattcattttgagttaattaaaattccatttgcaaaacactattttaatcgctgacctaggtgtgacaaatttataataatttgtaaaagttcttagggatgtctgggaacagtttcacaccatagaaaaataatttctgtagctagatagtaaattcagttttttcagccatttatagttaatgaaaatctgccttttaaattctgcttgtgagccattccaagaacaaaaacaatgtaacaaaacaaagttaaagtattgccataacctttttcaccaaagttggaacaacaacagaaaaatttaatagactttttgactcaaaaaaagatagaaggaacagataattatgaagtttcagccttttacatagtgaaatatattaagatttagctgtactttgtatgtttgctagagttgtacaatatcttatttctaagaatcattttgaaattcagaaggcattgatttctgatacattttactggaaaatgtgacacatttaccacatatgcagtataaaaactaaatgtgtgtaacacacagattgtgctcgtcatatttctcaaatatttttcctaactttcaagattttttcctaagtttcaaaggttagcttgtttgtttcaaagcaatttccaagtaaggtttttgaaaactgtaaatattaaaagatttaaaatgacagttttcatataatttaaggtaacaagactttctttgacttgcagactaatcctaaaacgaatggaagacttaacaaaactgcaaaatacaggacattttgtatttctgatcttaatgaactcatgtataaaataataatcttctcatttccccaattactacaggatttaaaataaaatacccttaacctattaattttggttagcatagttctatactgcatttattctattttatgcacatagtttggaaatgtgaaaggtaactaacagttttaatctacaactgttttgagacttttgaaatccataaaatagctaatgttatgtgctctaaaaatcctaatatttaaaatcgtcataaccctctgcatgccacaatgacatatacctaaggccaacttaaaaagagaaataatgcactcattaaataacagcaacaatgtaatgatacatgaaatgggctatacaatgacgtttcatgaagcagcacctgcttgtcataaggcattatgaaagaagattaaccttacttacacattacttttatcagaagtaaatgtgatcagctgccaacattttgaatggttgggaatctaacttcagttcaagaggtcacatacattttcaatctggagggctaacatgccttccttgtgcaattggtagactacacggacagatgcttagaatgtctacaattatattgtgctctaatgttacagaataattggaattcttggcaaaaggacttgcacactcaagaatgaactttttttcacacaaaaagcttatcaagaacaagacagtggctcaaaaaccacttttctaaatatacttccatacaaaataatttcaagatataattattagtttcttgtagagtacgctatttaaacaagaataaaagagtaagtatgtgaaaactgcaacaccacaaaaattgagccattttactagtgtaattaaacattagaacaatcttggaacaggcaagcaaaatattcagaagggtgaatcatggcggcacagctaactgatttttaccatgacttgcacactttgagacaacacaaataccttatgcagatggttcagtagcagaatggcacttggtttgctcctaatagaaacaacatgaatgcaactgacaatttagagatagacaatggccttatttgcatgctgaaaatctggttgtgttcctctagtccacacaccgttaactgtgcaatctgttgacgagtaaacaaatagtgcaggattcatctcagtgaggtctgggccccttggtctaaccgaaatcaattcttggtcgatactgcagtaccatagggtatgactgatacaaagggccatcctgagagcagacttgcgaagctgagcagttcagacaccgaaagttttcgcctcttagtcgccatcttgtcatgtagatgaattccatagtatgatccttccccataatttcaccattgcacagcacatccaactcataagaacttggaagttttagttttaaacttagaaattttttaatagttcccacagttacacgtgtagaacatcgaatgaatttcttcattaaaccctttactacattgtcccctgattgcccattatttcgtaaacaatctagacagatagcaatttgtgggtcacttctgtgataatctttatcatcttcattttcatcaccttcttcatctactttcggtttgtcagcttttgaagtatcatcttgtccattttcttgaggcttatttttcttccaaaattcagattcacgctcaagttcttgttctcgtagtccagggaccagcttaaatataatttcctctaatgtattgtccaacctcaacatttctaatggatttgtctcatgaacttggttgccacaccttgggcaatcattgctatcttcaaagtgctgaacaatacaagtcttacagaatgtatggaggcattccgtcactgttgttggcttgatcagataccctttacagatatagcaggtaatgtaaggattaaaatctttcaccaagtgtttcctttgggtagccattcgtggctagtgaagactggctttagtagtctgggcaaagaggggtcctaagtagatgaaagtctgatcccaggagctggtgtgtcgttcccagtaggatgtcctgaggcatgagaactagcatccagatttatcatgagatcgttgatcatcactccttttggtggttccgctttcccatgtcttgctctcgagaggccacgatccgggcgggccgcgcggggcgcgtggtgcgcgagcgcgcgcgcgtggggcggtaggtgagggagccc

SEQ ID NO: 15710 - RNA, 4981 nt, Homo sapiens
  source 1..4981: mol_type = other RNA
gctgggattacaggcatgagccactgtgcccggcctagagttgctttttaaggggaaaaaaaccacaggtccttatgaaatattttgaatatagagaaagcacttacttatataaatcccatagaatgaagtcttttctatacaagtaagtgtgttggcacttttaccaaagtctgcctttaataaaatttctcatattatgaataatacaggagctaaatctaagcttaattttagttaacactgcctccatgaaataaaaaccctctcaaattaaaaatctgaactttcttttcaaagtatgtatttctctcacttttcatgcagaggaaggctatttgttgtgtttacctctttctcatctttgaggatttagatttactaagatctgttagatgatgctgaaaaacaatgaacatatttgaaaggaagtgtgttctgattattgcaagaaaagcctgcatttgactgatctcaccaagaaaattcagtttaaagcctttctttggtgatattttagcaattaatcaaggttattgcctaactatataaaattaaattgcaatctaaaaatttccaacctccaaactgttaaaaccgtctctccaacatggttattaatttactgtaaaatgtctttggtgatatctatattcttatgaaaatcttccaaaaaaattaacttacaagagcctatttagatatgaaaccattcataagagacaggtacagataactcaaactttatgcagtaaatttaaaacagaaatgcactttagtaatgaggcactttctcttaaatatttcagtaaagctaaacagttcacaatattatataacacactttttttccttaaataatcagtttaaatttagattacatttgagtgtgtaatgtagttgagcaaagtcattacgtttataaaatgtggcacattactatgggatagatgtttaatgtataaagaaataatatactcctctaagagtagttaaaaggcattacccaagttacctgtactccagactgagtattacctcatcaatgagcattttagtttattttttcatactttgtaaagctgttttgctaatctagagaaaaggccatacatattttgatttctctattaactgatgtgattacttcaattaaagtaatgtttataaaccacagtcattctttatatctaagttcccttgacccttttatacttataatttctaaggcagataaaagagataacaaaatcttttatggaagtaaaggtctttcagtttattgcttaagaaacaacagattaaagaaaacttttagttttagtctctgatgttacagattcagatgattcctataggttatttaaagaattcattttatcattttataagcaccctaaatttataaagctaaccacaaaagttgcctgtacattttttctatacctagtttcttgcaaattctacaatctgacttaagggataattaacggggaatacagtgtattactagacatgaaagtagtcctatccttagaaagctgtagttgaatataccaaaataagtcagttgaagaaatctgtgattctagtagtaataccatatcacttaggaccatcaaaaaaatgtgtacctttctccaaacgacaactgatgcctttctttatgtaagcttttcacgtgttttggcacatattccattgcatttcaataaaaatgttaatgcattatcagtaaataaaagaattctatataaaactattctcagtttcataattgcttcctatatatttccttggaaaatagtgaaattacatatgacaaggcaaccagccaaatttaaagagattttgtagataaaattcatttatgaccattaagttttggctggggggccaaaacatcaaagtctcacttgtgatttttaaaatgcactcttaattcattttgagttaattaaaattccatttgcaaaacactattttaatcgctgacctaggtgtgacaaatttataataatttgtaaaagttcttagggatgtctgggaacagtttcacaccatagaaaaataatttctgtagctagatagtaaattcagttttttcagccatttatagttaatgaaaatctgccttttaaattctgcttgtgagccattccaagaacaaaaacaatgtaacaaaacaaagttaaagtattgccataacctttttcaccaaagttggaacaacaacagaaaaatttaatagactttttgactcaaaaaaagatagaaggaacagataattatgaagtttcagccttttacatagtgaaatatattaagatttagctgtactttgtatgtttgctagagttgtacaatatcttatttctaagaatcattttgaaattcagaaggcattgatttctgatacattttactggaaaatgtgacacatttaccacatatgcagtataaaaactaaatgtgtgtaacacacagattgtgctcgtcatatttctcaaatatttttcctaactttcaagattttttcctaagtttcaaaggttagcttgtttgtttcaaagcaatttccaagtaaggtttttgaaaactgtaaatattaaaagatttaaaatgacagttttcatataatttaaggtaacaagactttctttgacttgcagactaatcctaaaacgaatggaagacttaacaaaactgcaaaatacaggacattttgtatttctgatcttaatgaactcatgtataaaataataatcttctcatttccccaattactacaggatttaaaataaaatacccttaacctattaattttggttagcatagttctatactgcatttattctattttatgcacatagtttggaaatgtgaaaggtaactaacagttttaatctacaactgttttgagacttttgaaatccataaaatagctaatgttatgtgctctaaaaatcctaatatttaaaatcgtcataaccctctgcatgccacaatgacatatacctaaggccaacttaaaaagagaaataatgcactcattaaataacagcaacaatgtaatgatacatgaaatgggctatacaatgacgtttcatgaagcagcacctgcttgtcataaggcattatgaaagaagattaaccttacttacacattacttttatcagaagtaaatgtgatcagctgccaacattttgaatggttgggaatctaacttcagttcaagaggtcacatacattttcaatctggagggctaacatgccttccttgtgcaattggtagactacacggacagatgcttagaatgtctacaattatattgtgctctaatgttacagaataattggaattcttggcaaaaggacttgcacactcaagaatgaactttttttcacacaaaaagcttatcaagaacaagacagtggctcaaaaaccacttttctaaatatacttccatacaaaataatttcaagatataattattagtttcttgtagagtacgctatttaaacaagaataaaagagtaagtatgtgaaaactgcaacaccacaaaaattgagccattttactagtgtaattaaacattagaacaatcttggaacaggcaagcaaaatattcagaagggtgaatcatggcggcacagctaactgatttttaccatgacttgcacactttgagacaacacaaataccttatgcagatggttcagtagcagaatggcacttggtttgctcctaatagaaacaacatgaatgcaactgacaatttagagatagacaatggccttatttgcatgctgaaaatctggttgtgttcctctagtccacacaccgttaactgtgcaatctgttgacgagtaaacaaatagtgcaggattcatctcagtgaggtctgggccccttggtctaaccgaaatcaattcttggtcgatactgcagtaccatagggtatgagttttcgcctcttagtcgccatcttgtcatgtagatgaattccatagtatgatccttccccataatttcaccattgcacagcacatccaactcataagaacttggaagttttagttttaaacttagaaattttttaatagttcccacagttacacgtgtagaacatcgaatgaatttcttcattaaaccctttactacattgtcccctgattgcccattatttcgtaaacaatctagacagatagcaatttgtgggtcacttctgtgataatctttatcatcttcattttcatcaccttcttcatctactttcggtttgtcagcttttgaagtatcatcttgtccattttcttgaggcttatttttcttccaaaattcagattcacgctcaagttcttgttctcgtagtccagggaccagcttaaatataatttcctctaatgtattgtccaacatgtatggaggcattccgtcactgttgttggcttgatcagataccctttacagatatagcaggtaatgtaaggattaaaatctttcaccaagtgtttcctttgggtagccattcgtggctagtgaagactggctttagtagtctgggcaaagaggggtcctaagtagatgaaagtctgatcccaggagctggtgtgtcgttcccagtaggatgtcctgaggcatgagaactagcatccagatttatcatgagatcgttgatcatcactccttttggtggttccgctttcccatgtccagcggccgccaccgccgccgctcctcgcccgccagcgcgccggcctcagagtgaaggaaagtgaaacagaaacagcacccgccgcggcctggccggtccccgcgccccgtctgctctccccctgcaggcgggagcgcgccggctctgtggggccactcggctcaggcccgacagggcgcggcgggcctcggggcccaggtccggtgccgcctccaagggcaactccacccacttccaaccggcggcaccgcccgccccgcc

SEQ ID NO: 15711 - RNA, 5082 nt, Homo sapiens
  source 1..5082: mol_type = other RNA
gctgggattacaggcatgagccactgtgcccggcctagagttgctttttaaggggaaaaaaaccacaggtccttatgaaatattttgaatatagagaaagcacttacttatataaatcccatagaatgaagtcttttctatacaagtaagtgtgttggcacttttaccaaagtctgcctttaataaaatttctcatattatgaataatacaggagctaaatctaagcttaattttagttaacactgcctccatgaaataaaaaccctctcaaattaaaaatctgaactttcttttcaaagtatgtatttctctcacttttcatgcagaggaaggctatttgttgtgtttacctctttctcatctttgaggatttagatttactaagatctgttagatgatgctgaaaaacaatgaacatatttgaaaggaagtgtgttctgattattgcaagaaaagcctgcatttgactgatctcaccaagaaaattcagtttaaagcctttctttggtgatattttagcaattaatcaaggttattgcctaactatataaaattaaattgcaatctaaaaatttccaacctccaaactgttaaaaccgtctctccaacatggttattaatttactgtaaaatgtctttggtgatatctatattcttatgaaaatcttccaaaaaaattaacttacaagagcctatttagatatgaaaccattcataagagacaggtacagataactcaaactttatgcagtaaatttaaaacagaaatgcactttagtaatgaggcactttctcttaaatatttcagtaaagctaaacagttcacaatattatataacacactttttttccttaaataatcagtttaaatttagattacatttgagtgtgtaatgtagttgagcaaagtcattacgtttataaaatgtggcacattactatgggatagatgtttaatgtataaagaaataatatactcctctaagagtagttaaaaggcattacccaagttacctgtactccagactgagtattacctcatcaatgagcattttagtttattttttcatactttgtaaagctgttttgctaatctagagaaaaggccatacatattttgatttctctattaactgatgtgattacttcaattaaagtaatgtttataaaccacagtcattctttatatctaagttcccttgacccttttatacttataatttctaaggcagataaaagagataacaaaatcttttatggaagtaaaggtctttcagtttattgcttaagaaacaacagattaaagaaaacttttagttttagtctctgatgttacagattcagatgattcctataggttatttaaagaattcattttatcattttataagcaccctaaatttataaagctaaccacaaaagttgcctgtacattttttctatacctagtttcttgcaaattctacaatctgacttaagggataattaacggggaatacagtgtattactagacatgaaagtagtcctatccttagaaagctgtagttgaatataccaaaataagtcagttgaagaaatctgtgattctagtagtaataccatatcacttaggaccatcaaaaaaatgtgtacctttctccaaacgacaactgatgcctttctttatgtaagcttttcacgtgttttggcacatattccattgcatttcaataaaaatgttaatgcattatcagtaaataaaagaattctatataaaactattctcagtttcataattgcttcctatatatttccttggaaaatagtgaaattacatatgacaaggcaaccagccaaatttaaagagattttgtagataaaattcatttatgaccattaagttttggctggggggccaaaacatcaaagtctcacttgtgatttttaaaatgcactcttaattcattttgagttaattaaaattccatttgcaaaacactattttaatcgctgacctaggtgtgacaaatttataataatttgtaaaagttcttagggatgtctgggaacagtttcacaccatagaaaaataatttctgtagctagatagtaaattcagttttttcagccatttatagttaatgaaaatctgccttttaaattctgcttgtgagccattccaagaacaaaaacaatgtaacaaaacaaagttaaagtattgccataacctttttcaccaaagttggaacaacaacagaaaaatttaatagactttttgactcaaaaaaagatagaaggaacagataattatgaagtttcagccttttacatagtgaaatatattaagatttagctgtactttgtatgtttgctagagttgtacaatatcttatttctaagaatcattttgaaattcagaaggcattgatttctgatacattttactggaaaatgtgacacatttaccacatatgcagtataaaaactaaatgtgtgtaacacacagattgtgctcgtcatatttctcaaatatttttcctaactttcaagattttttcctaagtttcaaaggttagcttgtttgtttcaaagcaatttccaagtaaggtttttgaaaactgtaaatattaaaagatttaaaatgacagttttcatataatttaaggtaacaagactttctttgacttgcagactaatcctaaaacgaatggaagacttaacaaaactgcaaaatacaggacattttgtatttctgatcttaatgaactcatgtataaaataataatcttctcatttccccaattactacaggatttaaaataaaatacccttaacctattaattttggttagcatagttctatactgcatttattctattttatgcacatagtttggaaatgtgaaaggtaactaacagttttaatctacaactgttttgagacttttgaaatccataaaatagctaatgttatgtgctctaaaaatcctaatatttaaaatcgtcataaccctctgcatgccacaatgacatatacctaaggccaacttaaaaagagaaataatgcactcattaaataacagcaacaatgtaatgatacatgaaatgggctatacaatgacgtttcatgaagcagcacctgcttgtcataaggcattatgaaagaagattaaccttacttacacattacttttatcagaagtaaatgtgatcagctgccaacattttgaatggttgggaatctaacttcagttcaagaggtcacatacattttcaatctggagggctaacatgccttccttgtgcaattggtagactacacggacagatgcttagaatgtctacaattatattgtgctctaatgttacagaataattggaattcttggcaaaaggacttgcacactcaagaatgaactttttttcacacaaaaagcttatcaagaacaagacagtggctcaaaaaccacttttctaaatatacttccatacaaaataatttcaagatataattattagtttcttgtagagtacgctatttaaacaagaataaaagagtaagtatgtgaaaactgcaacaccacaaaaattgagccattttactagtgtaattaaacattagaacaatcttggaacaggcaagcaaaatattcagaagggtgaatcatggcggcacagctaactgatttttaccatgacttgcacactttgagacaacacaaataccttatgcagatggttcagtagcagaatggcacttggtttgctcctaatagaaacaacatgaatgcaactgacaatttagagatagacaatggccttatttgcatgctgaaaatctggttgtgttcctctagtccacacaccgttaactgtgcaatctgttgacgagtaaacaaatagtgcaggattcatctcagtgaggtctgggccccttggtctaaccgaaatcaattcttggtcgatactgcagtaccatagggtatgagttttcgcctcttagtcgccatcttgtcatgtagatgaattccatagtatgatccttccccataatttcaccattgcacagcacatccaactcataagaacttggaagttttagttttaaacttagaaattttttaatagttcccacagttacacgtgtagaacatcgaatgaatttcttcattaaaccctttactacattgtcccctgattgcccattatttcgtaaacaatctagacagatagcaatttgtgggtcacttctgtgataatctttatcatcttcattttcatcaccttcttcatctactttcggtttgtcagcttttgaagtatcatcttgtccattttcttgaggcttatttttcttccaaaattcagattcacgctcaagttcttgttctcgtagtccagggaccagcttaaatataatttcctctaatgtattgtccaacctcaacatttctaatggatttgtctcatgaacttggttgccacaccttgggcaatcattgctatcttcaaagtgctgaacaatacaagtcttacagaatgtatggaggcattccgtcactgttgttggcttgatcagataccctttacagatatagcaggtaatgtaaggattaaaatctttcaccaagtgtttcctttgggtagccattcgtggctagtgaagactggctttagtagtctgggcaaagaggggtcctaagtagatgaaagtctgatcccaggagctggtgtgtcgttcccagtaggatgtcctgaggcatgagaactagcatccagatttatcatgagatcgttgatcatcactccttttggtggttccgctttcccatgtccagcggccgccaccgccgccgctcctcgcccgccagcgcgccggcctcagagtgaaggaaagtgaaacagaaacagcacccgccgcggcctggccggtccccgcgccccgtctgctctccccctgcaggcgggagcgcgccggctctgtggggccactcggctcaggcccgacagggcgcggcgggcctcggggcccaggtccggtgccgcctccaagggcaactccacccacttccaaccggcggcaccgcccgccccgccgccc

SEQ ID NO: 15712 - RNA, 4997 nt, Homo sapiens
  source 1..4997: mol_type = other RNA
gctgggattacaggcatgagccactgtgcccggcctagagttgctttttaaggggaaaaaaaccacaggtccttatgaaatattttgaatatagagaaagcacttacttatataaatcccatagaatgaagtcttttctatacaagtaagtgtgttggcacttttaccaaagtctgcctttaataaaatttctcatattatgaataatacaggagctaaatctaagcttaattttagttaacactgcctccatgaaataaaaaccctctcaaattaaaaatctgaactttcttttcaaagtatgtatttctctcacttttcatgcagaggaaggctatttgttgtgtttacctctttctcatctttgaggatttagatttactaagatctgttagatgatgctgaaaaacaatgaacatatttgaaaggaagtgtgttctgattattgcaagaaaagcctgcatttgactgatctcaccaagaaaattcagtttaaagcctttctttggtgatattttagcaattaatcaaggttattgcctaactatataaaattaaattgcaatctaaaaatttccaacctccaaactgttaaaaccgtctctccaacatggttattaatttactgtaaaatgtctttggtgatatctatattcttatgaaaatcttccaaaaaaattaacttacaagagcctatttagatatgaaaccattcataagagacaggtacagataactcaaactttatgcagtaaatttaaaacagaaatgcactttagtaatgaggcactttctcttaaatatttcagtaaagctaaacagttcacaatattatataacacactttttttccttaaataatcagtttaaatttagattacatttgagtgtgtaatgtagttgagcaaagtcattacgtttataaaatgtggcacattactatgggatagatgtttaatgtataaagaaataatatactcctctaagagtagttaaaaggcattacccaagttacctgtactccagactgagtattacctcatcaatgagcattttagtttattttttcatactttgtaaagctgttttgctaatctagagaaaaggccatacatattttgatttctctattaactgatgtgattacttcaattaaagtaatgtttataaaccacagtcattctttatatctaagttcccttgacccttttatacttataatttctaaggcagataaaagagataacaaaatcttttatggaagtaaaggtctttcagtttattgcttaagaaacaacagattaaagaaaacttttagttttagtctctgatgttacagattcagatgattcctataggttatttaaagaattcattttatcattttataagcaccctaaatttataaagctaaccacaaaagttgcctgtacattttttctatacctagtttcttgcaaattctacaatctgacttaagggataattaacggggaatacagtgtattactagacatgaaagtagtcctatccttagaaagctgtagttgaatataccaaaataagtcagttgaagaaatctgtgattctagtagtaataccatatcacttaggaccatcaaaaaaatgtgtacctttctccaaacgacaactgatgcctttctttatgtaagcttttcacgtgttttggcacatattccattgcatttcaataaaaatgttaatgcattatcagtaaataaaagaattctatataaaactattctcagtttcataattgcttcctatatatttccttggaaaatagtgaaattacatatgacaaggcaaccagccaaatttaaagagattttgtagataaaattcatttatgaccattaagttttggctggggggccaaaacatcaaagtctcacttgtgatttttaaaatgcactcttaattcattttgagttaattaaaattccatttgcaaaacactattttaatcgctgacctaggtgtgacaaatttataataatttgtaaaagttcttagggatgtctgggaacagtttcacaccatagaaaaataatttctgtagctagatagtaaattcagttttttcagccatttatagttaatgaaaatctgccttttaaattctgcttgtgagccattccaagaacaaaaacaatgtaacaaaacaaagttaaagtattgccataacctttttcaccaaagttggaacaacaacagaaaaatttaatagactttttgactcaaaaaaagatagaaggaacagataattatgaagtttcagccttttacatagtgaaatatattaagatttagctgtactttgtatgtttgctagagttgtacaatatcttatttctaagaatcattttgaaattcagaaggcattgatttctgatacattttactggaaaatgtgacacatttaccacatatgcagtataaaaactaaatgtgtgtaacacacagattgtgctcgtcatatttctcaaatatttttcctaactttcaagattttttcctaagtttcaaaggttagcttgtttgtttcaaagcaatttccaagtaaggtttttgaaaactgtaaatattaaaagatttaaaatgacagttttcatataatttaaggtaacaagactttctttgacttgcagactaatcctaaaacgaatggaagacttaacaaaactgcaaaatacaggacattttgtatttctgatcttaatgaactcatgtataaaataataatcttctcatttccccaattactacaggatttaaaataaaatacccttaacctattaattttggttagcatagttctatactgcatttattctattttatgcacatagtttggaaatgtgaaaggtaactaacagttttaatctacaactgttttgagacttttgaaatccataaaatagctaatgttatgtgctctaaaaatcctaatatttaaaatcgtcataaccctctgcatgccacaatgacatatacctaaggccaacttaaaaagagaaataatgcactcattaaataacagcaacaatgtaatgatacatgaaatgggctatacaatgacgtttcatgaagcagcacctgcttgtcataaggcattatgaaagaagattaaccttacttacacattacttttatcagaagtaaatgtgatcagctgccaacattttgaatggttgggaatctaacttcagttcaagaggtcacatacattttcaatctggagggctaacatgccttccttgtgcaattggtagactacacggacagatgcttagaatgtctacaattatattgtgctctaatgttacagaataattggaattcttggcaaaaggacttgcacactcaagaatgaactttttttcacacaaaaagcttatcaagaacaagacagtggctcaaaaaccacttttctaaatatacttccatacaaaataatttcaagatataattattagtttcttgtagagtacgctatttaaacaagaataaaagagtaagtatgtgaaaactgcaacaccacaaaaattgagccattttactagtgtaattaaacattagaacaatcttggaacaggcaagcaaaatattcagaagggtgaatcatggcggcacagctaactgatttttaccatgacttgcacactttgagacaacacaaataccttatgcagatggttcagtagcagaatggcacttggtttgctcctaatagaaacaacatgaatgcaactgacaatttagagatagacaatggccttatttgcatgctgaaaatctggttgtgttcctctagtccacacaccgttaactgtgcaatctgttgacgagtaaacaaatagtgcaggattcatctcagtgaggtctgggccccttggtctaaccgaaatcaattcttggtcgatactgcagtaccatagggtatgagttttcgcctcttagtcgccatcttgtcatgtagatgaattccatagtatgatccttccccataatttcaccattgcacagcacatccaactcataagaacttggaagttttagttttaaacttagaaattttttaatagttcccacagttacacgtgtagaacatcgaatgaatttcttcattaaaccctttactacattgtcccctgattgcccattatttcgtaaacaatctagacagatagcaatttgtgggtcacttctgtgataatctttatcatcttcattttcatcaccttcttcatctactttcggtttgtcagcttttgaagtatcatcttgtccattttcttgaggcttatttttcttccaaaattcagattcacgctcaagttcttgttctcgtagtccagggaccagcttaaatataatttcctctaatgtattgtccaacctcaacatttctaatggatttgtctcatgaacttggttgccacaccttgggcaatcattgctatcttcaaagtgctgaacaatacaagtcttacagaatgtatggaggcattccgtcactgttgttggcttgatcagataccctttacagatatagcaggtaatgtaaggattaaaatctttcaccaagtgtttcctttgggtagccattcgtggctagtgaagactggctttagtagtctgggcaaagaggggtcctaagtagatgaaagtctgatcccaggagctggtgtgtcgttcccagtaggatgtcctgaggcatgagaactagcatccagatttatcatgagatcgttgatcatcactccttttggtggttccgctttcccatgtctgtagtggcccgaccttggcaaggagaaattcgaaacttctcaggccggagacttcgaatcgtacagcctctgagggggcaccttctccccccacagacggaggaagcgtgcccttgaatagatggaaggcagctcgaatgtcagtatgcctccctggcgatggtcaagtccaggcttccc

SEQ ID NO: 15713 - RNA, 4119 nt, Homo sapiens
  source 1..4119: mol_type = other RNA
gctgggattacaggcatgagccactgtgcccggcctgggagctcattctggaaattactactttttgtactaactttgtgtgccatgtactctgggctttatgtggcttcctctcccccatcaccccttattctgaacagctgtgaggtagataccattatctgcactttatataaatacttagtcttctacggctaagagcagggttcaaacccaggtattccaacctgtgctatttggagtatattaatccacctgtctttactaaaggtgaaaacttttgcatgtggttcaatagtcagggagaagttagaaaaaaagtaatggaagaataatcatgaatttgtatgcttctatacattaactagctctttctccctttttccagagttctcttggaacggttgattgtaaataggccacatccttggggtcttcttattaccttcattgagctgattaaaaacccagcgtttaagttctggaaccatgaatttgtacactgtgccccagaaatcgaaaagtgagttcaaagtaatttttaattgtctaggaatgagactggagactgaaaaccatctgtctctaggttgggtcagctgaatgagatgcaaggtattgttaggcctactctttaatcagagatttgtaactgtcttcatccttcaggttattccagtcggtcgcacagtgctgcatgggacagaagcaggcccagcaagtaatggaagggacaggtgccagttagacgaaactgcatctctgttgtacgtgtcagtctagaggtctcactgcaccgagttcataaactgactgaagaatcctttcagctcttcctgactttcccagccctttggtttgtgggtatctgccccaactactgttgggatcagcctcctgtcttatgtgggcacgttccaaagtttaaatgcatttttttgactcttggccaaaatttagaagatgctgtgaatatcattttgaacttgtgtaaatacatgaaagagaaaacctttgtctggaacttcttggctttgtgcaagctgtgtccaaggcaagtacataaactggtaccttgtaatgaagaggcagctgatgccatgcacttgtctgagggcatagctccatgtcttctgacattcctggtgtcccaaagaatagcaaaaagccagtttgaatattatgtaacttatttttttaatgtggacaggggaccttgaaaatcactaagttattaaaaatgtggatgtgctagaattggatatgtccaggaacatgggaagggctcactattggaatcccatgagtttccattttgtctctacccaaacgtattccaaagctgactgcatttgtaccatcttatttcttttggggattatacacctcagccgcctgagatgggggtcagctctttatataaagggaaaccagaccaggcctaaagcccacccctaccctcacccccccaatcctctcctgaaacttaaaaacagtgggaatataggaaagggaaccaaatctcattaattaattgttctcccccattaccccactgaatgaatggccatacaggctaagctgaataatgacaaagttgaaaggaccaatacagccccttttataaggattttgaatgttttgcaaatgtattggtccctgtgttgtattttgtagccttttcctgggcttcagctcccctacttcttgtatgtgtatgcatactgtagctaaccattaaagtcatgacacacacatgagtccactgtgcctttctcagtagcagcagccagtgctggtggtgaggaggaaaagtggacaatccagccctgcagaccttggggccatggggaaccaccaactaacttcttgctgaatgattgattgattgattgataggtcattcctactactaagctggcatgtttaaggaaattgtatttttcttcctatttatttcaacactggacaaatgctggagcaggtttatctggttaagctgagtttaaaatacccagttttaatatccttttcccccaggtattttttttttttttttaaagaaaatgagtagatacgtatttaaaaacttaacccacttaaaatttgccttacctttcatgactgtcaagttttatggccagagaggacaaaacagttcaaaattaaataattgaagtcctccttgagtgatgtcttagggtttattccctgagaggtggtttgtgccatctagactgaactttgggtaactatcgagtaccagttacacagcttattaaatccagagtcttttcaataaaggttaagtgacttcctcaaactagacttagatttaaaccaggggtctacctccaaagtctattattaaatgctgaaacacaacaagacttacttattactaccgtatgtccactggctttggttaaaactgagaacaaaacatctgtaacatgctttaagtaacaattagcagtgattcccaagtctgctgttctcaatcctaaaacacatcacccttacctgagttaatcctagcacaccaactttgctacttttcctcttggtgtttagtaagcaaaagaaagatccaaattttcctctttttcaaacatcaatgagtattagcttagaataaagttcttattgctgttccttcagggaacagggaaactgctaacttgtcagctccaacaactgatgtaagatcatcttctgaccatagcgaacctgtaaggcttgctgttccctccagctgagtttcgcatagacttccttattactgagtaaaccttggtcagtttttaagtctgtggcataggtctgcaaagtcagtagaacactgttttgaagcagctgtctccacgatgctttgagcttgggaatatttgtgatcgtcaggctgccctcttcccttttatcatctccccctccatcctggtctttaagctctctgaactcctcagcaggcatgcacagtacctttagtgtggtggtcagctcctcttcagtcagcacctcctccctccctatcacaaaggctccctcttcccctaccatctccagtttgcataggaaatcccagcgctcgtacactaggtgcctttcagcttcagtttttgttccctgtaatgctgcctcacgaactgtcaccatctgaatgtcagctgtgtcatctgtgttgtcaggatatggttcaacaaaaccgtacatatgaatcagttgccagttagccatttgcccataagtgttgaaaatctcatggcctttaggaatgggctgagtggctaccatccgaagacaattcgcagagtattctagattggcgttgtgattggctaagtggtttagtatgtctgcagcaggcaccatcacgggggagttgggctccttttcatcctcttcttcctccagtggttcctgaaagctataggccatcacaagggccaccagctggtggtagagttctagggagcgaaccctgaggctgaagagatcggggtgggcttccatgaagggcagcacgatggactggtactcgctgcggatgttggccaaatccttctccacggcctcaggtacgcctgtgccctggagcaggcaccggcgctcctcctctggccagaacatcgggtgctccaagcggcccagctcgggccagagcgcaaagtagggcctccagcgtgaggccggggcctgcagctcgtggagcagcgccagcagcagtggcacccagcccgactggctctgcagcgcaactcgctctcgctccagcaggccgccgatggagcaggtgtgctgcgacaggagcgcggcccgcggcaccacgaacaacagctctccggcctgcacgctctcccgggccaccatgccgtagccggccaccgtgccctgccggctgaccgccacctgagcaggagggctggtcagggcagcccgcgccccgccgcgggtcctccgcccgccggctcgctcgctcaccttgggactcagctccagccccacccgccggcaccagctcaggaagcaggccacaggatccaggtcgccgccgtccacgggccccgccacccgtggacgcttcgcctgggtcgccatggtctaagagcgcgtttcctc

SEQ ID NO: 15714 - RNA, 3967 nt, Homo sapiens
  source 1..3967: mol_type = other RNA
gctgggattacaggcatgagccactgtgcccggcctgggagctcattctggaaattactactttttgtactaactttgtgtgccatgtactctgggctttatgtggcttcctctcccccatcaccccttattctgaacagctgtgaggtagataccattatctgcactttatataaatacttagtcttctacggctaagagcagggttcaaacccaggtattccaacctgtgctatttggagtatattaatccacctgtctttactaaaggtgaaaacttttgcatgtggttcaatagtcagggagaagttagaaaaaaagtaatggaagaataatcatgaatttgtatgcttctatacattaactagctctttctccctttttccagagttctcttggaacggttgattgtaaataggccacatccttggggtcttcttattaccttcattgagctgattaaaaacccagcgtttaagttctggaaccatgaatttgtacactgtgccccagaaatcgaaaagtgagttcaaagtaatttttaattgtctaggaatgagactggagactgaaaaccatctgtctctaggttgggtcagctgaatgagatgcaaggtattgttaggcctactctttaatcagagatttgtaactgtcttcatccttcaggttattccagtcggtcgcacagtgctgcatgggacagaagcaggcccagcaagtaatggaagggacaggtgccagttagacgaaactgcatctctgttgtacgtgtcagtctagaggtctcactgcaccgagttcataaactgactgaagaatcctttcagctcttcctgactttcccagccctttggtttgtgggtatctgccccaactactgttgggatcagcctcctgtcttatgtgggcacgttccaaagtttaaatgcatttttttgactcttggccaaaatttagaagatgctgtgaatatcattttgaacttgtgtaaatacatgaaagagaaaacctttgtctggaacttcttggctttgtgcaagctgtgtccaaggcaagtacataaactggtaccttgtaatgaagaggcagctgatgccatgcacttgtctgagggcatagctccatgtcttctgacattcctggtgtcccaaagaatagcaaaaagccagtttgaatattatgtaacttatttttttaatgtggacaggggaccttgaaaatcactaagttattaaaaatgtggatgtgctagaattggatatgtccaggaacatgggaagggctcactattggaatcccatgagtttccattttgtctctacccaaacgtattccaaagctgactgcatttgtaccatcttatttcttttggggattatacacctcagccgcctgagatgggggtcagctctttatataaagggaaaccagaccaggcctaaagcccacccctaccctcacccccccaatcctctcctgaaacttaaaaacagtgggaatataggaaagggaaccaaatctcattaattaattgttctcccccattaccccactgaatgaatggccatacaggctaagctgaataatgacaaagttgaaaggaccaatacagccccttttataaggattttgaatgttttgcaaatgtattggtccctgtgttgtattttgtagccttttcctgggcttcagctcccctacttcttgtatgtgtatgcatactgtagctaaccattaaagtcatgacacacacatgagtccactgtgcctttctcagtagcagcagccagtgctggtggtgaggaggaaaagtggacaatccagccctgcagaccttggggccatggggaaccaccaactaacttcttgctgaatgattgattgattgattgataggtcattcctactactaagctggcatgtttaaggaaattgtatttttcttcctatttatttcaacactggacaaatgctggagcaggtttatctggttaagctgagtttaaaatacccagttttaatatccttttcccccaggtattttttttttttttttaaagaaaatgagtagatacgtatttaaaaacttaacccacttaaaatttgccttacctttcatgactgtcaagttttatggccagagaggacaaaacagttcaaaattaaataattgaagtcctccttgagtgatgtcttagggtttattccctgagaggtggtttgtgccatctagactgaactttgggtaactatcgagtaccagttacacagcttattaaatccagagtcttttcaataaaggttaagtgacttcctcaaactagacttagatttaaaccaggggtctacctccaaagtctattattaaatgctgaaacacaacaagacttacttattactaccgtatgtccactggctttggttaaaactgagaacaaaacatctgtaacatgctttaagtaacaattagcagtgattcccaagtctgctgttctcaatcctaaaacacatcacccttacctgagttaatcctagcacaccaactttgctacttttcctcttggtgtttagtaagcaaaagaaagatccaaattttcctctttttcaaacatcaatgagtattagcttagaataaagttcttattgctgttccttcagggaacagggaaactgctaacttgtcagctccaacaactgatgtaagatcatcttctgaccatagcgaacctgtaaggcttgctgttccctccagctgagtttcgcatagacttccttattactgagtaaaccttggtcagtttttaagtctgtggcataggtctgcaaagtcagtagaacactgttttgaagcagctgtctccacgatgctttgagcttgggaatatttgtgatcgtcaggctgccctcttcccttttatcatctccccctccatcctggtctttaagctctctgaactcctcagcaggcatgcacagtacctttagtgtggtggtcagctcctcttcagtcagcacctcctccctccctatcacaaaggctccctcttcccctaccatctccagtttgcataggaaatcccagcgctcgtacactaggtgcctttcagcttcagtttttgttccgcagagtattctagattggcgttgtgattggctaagtggtttagtatgtctgcagcaggcaccatcacgggggagttgggctccttttcatcctcttcttcctccagtggttcctgaaagctataggccatcacaagggccaccagctggtggtagagttctagggagcgaaccctgaggctgaagagatcggggtgggcttccatgaagggcagcacgatggactggtactcgctgcggatgttggccaaatccttctccacggcctcaggtacgcctgtgccctggagcaggcaccggcgctcctcctctggccagaacatcgggtgctccaagcggcccagctcgggccagagcgcaaagtagggcctccagcgtgaggccggggcctgcagctcgtggagcagcgccagcagcagtggcacccagcccgactggctctgcagcgcaactcgctctcgctccagcaggccgccgatggagcaggtgtgctgcgacaggagcgcggcccgcggcaccacgaacaacagctctccggcctgcacgctctcccgggccaccatgccgtagccggccaccgtgccctgccggctgaccgccacctgagcaggagggctggtcagggcagcccgcgccccgccgcgggtcctccgcccgccggctcgctcgctcaccttgggactcagctccagccccacccgccggcaccagctcaggaagcaggccacaggatccaggtcgccgccgtccacgggccccgccacccgtggacgcttcgcctgggtcgccatggtctaagagcgcgtttcctcgcgggccggcgcaccgcgcggtcacttcc

SEQ ID NO: 15715 - RNA, 3448 nt, Homo sapiens
  source 1..3448: mol_type = other RNA
gctgggattacaggcatgagccactgtgcccggcctgggcagtcgattttcaggaagccacttaatgttcagattcttttcttctctcccaggactttgcagatgctgctgttccctctgcctggagatgttcatctggcctgaatccaaaagtctgtccaagttacttctcttttccatgacagagttacaactatttgtctgtcccccttccccattagagtatatggtccccaaaggaaagccccatgccattcactcaccacctaatcatccccaacaactagtgggcaaacatgaaacacttttgttgaataatgtgtttcctttagcccagggattacaaagtcaaaggcttacaagggggaaggactagcaggtgtgctcggaggggactctagccaactggagagtaactggtgagaagacaatgacatgctcttagggtgtctgctactcagatcctctcagttaagtcccgtgcacaaaggtgggtcaggtctactgttgccagatcttcagatcattcaaaagttacccgaattctggattttcatgcaaatctcccaatttttaaaaatgttggcatcaaattcagaatgttttaaccagccacactgtgtgggccagggaaaacaggcccaaaggccaggtgaagctgcagttttcaactgctgccttggcctctcccagagccccttaagtcctaagaaggctcagtcaacacactggcactcgtttcatcccactggttgagaaagcaagtcttagcaaagtaatgggggagtcttaccaaaactgcaaaggaaaaaaatatgataccatgaaattagaaattcactgcatttgaaatgaaaatgacttatttctgtacttctataactcacaaatttagcagacatcatttagacatttttgtagtgcaacagatttaaatctggaatttcatggtttgtaaatcactatgtgatactagctataaccatgagcaatattacgggcagtaaatgttgatttctatttcgtttcttgaagttttgtgtggttcatttttaaagtgagattcaatttccttagctatagtcaaatgtaccctttaaacagcccaagaattgttataaatgacagctgctatcagttttcaaattttacaatattagggttgttaactatttcattctgaattaagctaacatttgttaccaagcaatgcatttatttggaaggataccagttaccagtcatcaaaagcttttgtatgttgaaaatgtaattttaatagttaattcttcatcttacataggagcacaataaaatacaccacaatctgaagaaactccagaattacgagaataagagtgaagaaaattcaaatgggctacaatatccattaccttaaactgcaagagacaaggttgcaacccgaaggttaacatttatgtatttatgactggctacatttatgacttaaaaataacaagaatcaggaattagatatggagagaggtgggaaagaacagttttgtgaggggaggaattcgtcaataaagaagaaaaattactgaattccaaattaaagaataaaacgagctcccacagcaaatactggagggatgaaagcaagaatcattaactgaggacttgatactctcaaagggataaacctttctgatgacacacaagctagatagttgagatctgctcatcaggtttataaggaagactcacaaatgcctcagcaaatcccaaatgatcagatcagtgtttcttaacacacatgaaaggttacagatgaaattttcagataagaaccaagaaaaatgtcataacccaaattttaggcaaaaatgtggcacaactgtgaaagtcctacatgtcagtcacaactgctatctttgctgtgactttcctgtacagtaatttttaaacattgtggcaagacaccaatgatcatctaatcagacaacacaaacacatttatttcaaattcctagaaggttaaaaaaaggtcagatactgatgctttatgcatgctcagggccagtttataaatactccattcagtactatcttaacacaaatctgcatcagtgaaaagaaactggcaaaatccacctcttgccattcaatttgtcagatggtgaagaccaagaaagaatgttccatcagtttcaattttaaaatacgattgtcaaattgggaaaatgaaataaacacagtaaaataaactgtacaaaggcaaagtagaataacaaaaaatattttactaaaacataagatttacagaagtttccagacaagccatacaaaatggtcacaagctttttttgaaggggggaatctacacttgacagcaatgttattagtgagggctgtgatgtttgtttaatgttcccattttggttccaacaatcaagcttgtccatctacagcgtctaaataaagttagacttggctagagcatattctaaagacctggttagctgcttttaaccaatgcaattagatcaccaaaaaagggggaaaggagcccataaaattaaactacctcccccctcaaaaataaaataaaataaaataaaataaaaacacccacacccctgcagctaacctgacaactaccttcattcacagtgctttatacttaaaccaggatgggggaaatgaataaaagcagggaggggccactgcttttaaacgtttcacaacaatccagatgatacttctagcctctgctcatgctttatgacagtgaatcaggacaagacatagatttgctaatgtgcatttaatcaccaaaggactgaagatgtctgggcttttttattctgtaatgtttctaagactgtgtccattaaatgcaaacaaagaggaggaagtcttggcagaacaggagaagtgatgcacacttgatgatcgtatcaatttaaatattattcatggcatatagcctagtccatgctctagctgtttctatggcttgggcttcgttggtcttccactgctccgctacatcatttgctaatggatcatctggattgggagcacttaacaaggcctggatcgatagcagaactgtgcggatctgcagtgctggggaccacttatctttcaaaatatctaaacatattcttcccaacttgtctacattaggatgataaattttggtcatgaaacgtactttaggggctgccattgggtattcttctggaaggaatagttcaagtttaaaagtccctccctcaaagggggaatcctgagggccagcaatgaccacatgaaaataacgggcgttgctctcatctggttcggctttgatgccaggaactggttctgccagcaaacgctgggtttccttgatgatcctgcggggcagcccggccatcttgtcagaacccgagttcggcctctggtctcgtctccggctcctctcgcctcacgcacgagt

SEQ ID NO: 15716 - RNA, 10199 nt, Homo sapiens
  source 1..10199: mol_type = other RNA
gctgggattacaggcatgagccactgtgcccggcctggtgttggatagttttatgttactggaaatacatgtgaactttgctcagagatgccaattagttattggaaacggtttgatctttttttccaaatctttgaagatttgttcagtggggccgccatagtaatacatggtctaggacttgccaggactgaggcaagacccctatgaatattctacctaatgccctattaattatggggatttctggtatagcccatggcaaccacctctattcatggttgtatgtgaacatgcactctcagtgagagtaatattgtccccaaaacgacagaaattagtttttttgggggggatgggagaagtgaagagaagaaaaatattctttttgtgtaaagcccagatatacgtatagtactaaagagatatgcagtgcatgtgcgatattaaaatttcagggcgggcgcagtggcttacgcctgtgataccagcgctttaggaggctgaggtgggcagatcatgagatccagagatcgagaccatcctggctaacacggtgaaaccttgcctccactaaaaatacaaaaaaaaaaaaaaaaaaaaaaattagctgggcatgttggcttgtgcctgtagtcccagctactcgggaggctgaggcaggagaatggcatgaaccctggaggcggagcttgcagtgagccaggatcgcgccactgcactccagcctgagcgacagagcaagactccgtctcaaaaataaaataaaattaaattaaattaaataaaaattaaaaaattcatagagaggtgactagaaaagatgtttaaaaagattccttgaggtcaataataattttttaaaggttgataaatgccgctgtaattcttttgagtgtttctttcccttgcctcaggtagtttcatgcactttgttacacactgaagggcgaccctctccagatttgcaaagttttctccaatgcagctctttcctcgccggtactctatcctgcaatctctagccaccttcgtgtacctgaactctcagcaacagctactccattcagagacttgctaggcttccttaagctatctatctccattgtcactgctgtctcaaattctctcaagttgtaagctgggatactcacagcacacatcttatgtttcctgtctttcagggattacattccgtgcctcatgtccagtgtactgaaaaccatagtttcatatattttgtctggtttgaggttgtttcatgcaggagggttagagggtaaatatgctccctattactccatcttagccagaagtaaaataagaaaaagaaatatatgtaagtataaacacacatacacatatatatatgtatgtatataacacacatgaatcatatcctaaagatttggaacaagaagtaaatttagctatcaattatgtttactcactgcagattaagatgaacattgtagattggagcatattatgggagcaaggcaacctgtagaattggtcaggaactagacatctcaggacctgcattctaacccatttttgtcagtaattatctgtgtaatgttttctcaaagcagtgaaggcctttgtgaattttgcaaaaatggggacaattatatgttttacctcattggcttgcttaaggagttaaaatgtgatatgagtcatacaaagtgctcatgcagtcacagaggttctattttaagggctttcttaaatttttaggtaccatcacaagctagctaagttagaaattttcatatcgcaaaatctaaaagttcatcttatgattttaaacatttttattcacagagcaaatgcaaccatgtgaacctcacattttaaaatatataatggcacaataaaatgcaaaaatataattttaggtcataacctataggcaataaactatgttatcattttgtaaaaaaaataccacaggaagtagtgcttcagtacattttcccgacgatatgattaatccataataaattctgctactactcctagtaatggcaactttatgtaaccttcttaaggttacatttgcacttaagtataccaacttaaaccgtgagtggctgttctgacaacacatcagcaatgaacttagcctgagctacatccattgggagtgatgtgaaggaagagaaaagcgttggactctatgatatttaatgtctttaccaatagaaaagctctgtaattcttagaattcaattttttaattaaaaaattggttctctctttacacataattgccaaaacagtgtttacaaatactttcatcttgccccagattggccaatgaggtagtaggttaaacagccaattcatcatgttttgatttaaaatgtgtccatatcattcttccccaaattcaagtatattttaataatccatttctgttacttatattatggattcaagaataaactaagcaaatggatcatttgtttgccttccagttatacatgaagaaattaatgttttattaaagaaaaaagccatcaaaatcaattttccatctgcactcttttatttgttgcaatactgtttataacagctaagatttggaaacaccctaagtgttcatcaacagatgaatgaagaaaatgtggttcacatacaaaatggagtactcttcagccataaaagagaatgagatcctgtcacttgcgacagcatggatggaactggaggtcattatgttaagtgaaataggccaggcatagaaagacaaacattgccatgttctcatttatttgtgggatctaaaaatcaaaacaacggaattcatggatatagagtagaaggatggttagtaaaggctgaaaaaagtagtagacagctgagataatggtggggcagaggtggggataggttaatgggtacaaaaaaagtagaaagaatgagtaaaacttactatatgatagcacaatagggtgactatagtcaataaaaacttaactgcatattttaaaatacagagtgtaatcaggttgtttgtaacacaaaggataaatgttgaggggatggataccccattctccatgatgtgcttatttcacagtgcatgcctgtatcaaaacatttcatgtactccataaatatatacacctagtatgtacacaaaaattaaaaaataaaaaagatttcccatcaaatattctttcagagaagatgtgaacaaagatccagaattattggtcagtctaggcaaacagtatcaaacagcctaatatgattttctcctctgctaaataatactgggaaggcaggaaggtgggcttctctatggattgaagttaagagagagaagtgccaggagttcagtccacgcatgacaacttactagtactgcctacttgaagagattagctcttacaaccttatctttgtctcatctataaaactgagggagcaggttaaaaaaatcttacatgttaatacatgacttatcctactccatgtctctattacaatgaaagatcatacacagtctggaagaaaatgttaaatttactgtgacttttcacagtaatagagacagagtaatagagacacggggtagaatatgtcacgtatcagtagtaactactatcaaagtatgttaagtttatgccgtaataatgacttttagtaaacaatgaagatttacagtgatttcctaaggtgaatttggacaaaaatattgagataataccactcaccagtgtcactattttacagagataagccttcaatgtcacatgaaccactctatttttaatattagaattctgaagtttttaagcatcagaatcttcagctttctcaaatgaagaatggtaattatatgctattttcttttttaatttgaagaaaaaagttgggaaattattatgcttttacttttatgttacaaaagggtgttacttgcaactagcatctatgtatctaaataacgtttagtgacttaattctctgcaacagtaaaaagtactcaatttagattttagtaagttgactgttagatggttgctctttggcagaagtttaaatatatatattcatagatatttttacatctagcaatcagtaaatatttatctctttttcttgcactttgcatttaataatttaaaaggaaaaatttaacagatgataaatatcaaaccaaaaaagtcaacaaatcttaataatctcaaaatatacaagggcaaagtgatacataaaccaatacagaatacatttgtctgcacatttttgcataaattttaaaaagcatataattctgtaattttaattttatagagctttccctaaaatattttttattttatttaaaaatgagtttattttcaaataagaagattaagtctaaaaatcagtgcaaaagattgatggtgatgatgtatcaatgcaatttgatgcatccgtttcgctgtcttgcaaaaggtgcagtgaccaatgggctgtctgtactctcaatacagatgtagtattctgagaagagatcatttgttaagagcggatttaagacagagagtgtattcattctttcaaaaataacacatacgaatttccataacaagatggaaattcatttacgtaacagtaacgctgaatcaatatattttcagcttgccctgatgtggaagaaatataccatctcattagtccttggtaggcagttggtatctggaatatgaagagtgtagcatcattgcttttatgtaattggtttattgaatccaaatggtggttccatgcattatcaaataaccactgcttcaatactagtccctggaactgtctccataaagttaattccaatcctttgctgtcttagtgtgtatgtaaaccttaatgagacatgttccagttaactgcacatattcaattttgggtaatctatgggaatttggccccatggtcataaacctgtgatcagactggcagatttaataaacatcatgtaaatgctaacttaacttggagtgaacagtcttcagtttacattccaaaagtgattagatgaaaggataatacacaatgatatttatgcctagagcagttcaaaatttagaaaaggaattagtgatcttcagttaagctatttttttaataaattgaaaagatgttctgtacaacataatagagtcataggaaatcaaaagcatatcagtaacaacttttagaaaaagaaatgaatgataaagaaaaacagatatgacctctcaatatcttggggaagtaagttaggatgatgtttcattcacgtcttaatgatataaataaaggataactctgtgtaagaagtattgtttgtatctggtggtaaatttagttaaaaacataatcacaagttacaaaaactgtaattacaaattacaaagaaaaacaggcagacaatcttgtattgacatcctcttgcatcttgttacctaccaatgttctgttccattataaaattcaatactaaaatttcatagctaacattcaatattaatttcaacattaaaatgtatcaaaatcattaaaaacagtcaattagaaaaagcaatacaccaaaaataatggtagtgtttccaggcttcaactgtgttgtattaaccatcacacaggagaataaaagggctgtgaattttagataggccacttggctctggattccaggactatggaaatgccagtgaaggtagtccaagaagcatttcttgttttataaatatcagcagaggaccaaaaaaagggatcccagatatgttttcaagtaacaaaaaacattaaagtgcaattttgtcttttacatctgaacaaaagttctgtcatttttaaaaaataaagtagggccacagctttatagccattttctcatctaaaaccccacaattattaacacagatcaaactgcagttttggaagagagcctttggacggggaaactactgaacagtgatgaatggccatacctaattcattgtttggaaattgatgtggaggactgtgtttcaccgagggagaaagggacctcccagaggctccgaggctgcaggtcttcagccaggtgacagcactgcacctgcttgtgtgcaccctgatggcaacagcagggaagtccacagtcacgatgatagagacagccacagctgccaatcagaagactcgctctttctggttttcatggactgcgttttgcacatcgagctcactgtttagagctgtcctagcactcttctttttttgagacttttgactcattttctttgcgtaactttctctgttgatagatgcgtatggctatggcagtgatgcaaagcaaaataaatatcaccactgctatcacacctccgatgacagcagagtctcttctgtctgcattaaccaagggctctccctcatccgctggtccagaacgacctgcgccccccgcgagtcggggagccagttcccgcgccggggagccggacgccgcccccgctgcgcagcgggccataggggccacgtggccgcggacggtgacccgggaggggccgctggggcgcagcgccgccttcaggggagcagcgcggccgaagcgcaccgccgagaggcagccagtgaagccactagtcgccgcccgccttgtgtccgggtccgcgccggcagcctctaaaacctttcccaatatgagagatttgacggcgttgaattctgtccctgaggacaagatgacttgtttctttgtgctctggttaacctctaccatgaccacagcttcttctctgttaatcttcacttggtgaagttgcccatcagccatgtttttaaaatcaaaggtaaatgcatcaggattttgatgtctatctagcttgtacctaatctgcaaacttccattgttggcgaggataactgaaaggtattcctcatagaaagagctcacatacagcaataagctcggagttcgtgtggttcggaagctcagtgtgatcatttctctggtcaatgttacatctctgtgtaatgaagaaacgagagagctggagttttcacttaaagtgtaatgttcttgaaaatggtatgtcattgaggagccagttgcaaaatatgcggaaatctcattggagcagaacggcccatcataggctgagaaggcacagtcacaggtgacccccctgcgtttctctctgcatctccctccattgcgacacaagtgtccataggtgctgcagtgtcctgcacaccctggctccactcctggcgtcactgtggctctttcttccagatccagggccaccccgttcaactgcagagaccgaatgcatcctagaaagcctctctgtctggtggccgttccaccaatgaagagctggctgttgagctgtaaacgaacgtgcccatcagcaggggcaggctgcatcttctgaggaagctgatcaacttgaagagacgctcctttaacatttctctctgccctcacgtggtgccactgattgtcattaaagggagtgggtgactgcaccgtgacctcacaaggtccattccccacatcgaaggaaaaggtcacttctgtgggagcacgcagctcaatcctgatgaaatctgtgatccccaggttctccataaacaccccggaggaaactgtggtcttaaaaaagaagcacacgtcagcagtgagttctccgtggaaagcagggaaatgaaggtatgaagtctcagtgttgaaggaagctgaattccagaatgactgatctccgcggcagagcagtggccccagtgtataagctgcttcggaatgtggtcggcctgcgtctgtcatcacaatctgagtgactggcaggtgctccttttgggaaaggactattgtgtcactagtccattcattccggccagcatcacagttgcagtaatactgagaatcaatgcagttcccctctaatccacaagtacacttttgagcatcaggcagagaacctccccaggaagtgtgtgtttcattggttcttccaacccaccagctcagtggggttccatctcgtgagtccgggcgccgcgccgtcccgcagcgcagagccagccgctgctcgcagcgctccgccaggttcaccgcggaccgcagctgccccgcgcccgctgcgtacgcgaaggacacagccgagcgcgggtgcccgctgggggcacctcggagggtcaccgcgtcggggccaccgtgctgcaccaccgtccacgcggcgtctgctgtcatattgcagtacacaagaaatggtcccagggggccacttccatctgcatcaatatagtaaagcccagacgggttccctcggtgcttgtgggcttcacaagactgctcgtagagagaggaatggcaggtctcgcccgtatagcctgtgcctagacagtcacaggagaaggtgtcccacgactgggaacactcgcccccatgctcacagtagctgggcaagcacctgtctgtgatgccgcaggagtctatctggaggtccctgaaactccccagcgccccctgctgtactaagatgggatccaccgctttgtcaccaatggtgatgagccttaggcagccctgaaaccctcccagggggcttttacatccagagccagagctgttgtccaggcagcctccaaaataataggtgtcacctgaatcaatgagcacagccaccaggggctgaacagctgtgtcatcgtccaccaccacattcatatggctccacttggcagagaaggacacagagtgccactgcccatcgtttaatccagcacctgctgtgacattccttggtgactgtcccggctggaagagactcagtttgagcttgccatccttaagaaagaggacgaaactccctgaaccacgtcgaagttcgccgaaaagcaaatgtcctgctctgttccacgttcgaaattgaaaagtgacagacactttgtcctccccagagttgcctggcagagccagataactcctggagctcagaaaagtcacagggacagtctgtggctgtggacatgagaaggacacatttcccatcatgaggatctgtggtttgtgtttcttggctaattcggtaacatccactccattataataaagattttctaaacacccatgaaagcttttacgtctgaatgcccgcgatcttccgggtgtcggaattcccccaaagctgatctcaaaattaagatccaagtaactggaatctccctttgcttggaaatgatgagtgtgtttgtccacggtgaagttgacctgcgtgtcgaggagctcgatgaggacggaatgccagtgctggtcgtccagcaggctgcccagggtgagggtcacaggagcaatagtggaaggcagcttagcattgcctgaattaagaaaaaagacaagctttcctttaattaattccagagtaatgtgatttccatgttgtccttctctgtgaagtagaattccattgctctgcatggctttaaatttcaaagaaataacgtctcttattggttttaaaggttttttatcaagtctatacagcagagcactttgtccatcaaaataaaccacctcagatttatatgcacatccgtacacttcgatccgcatcccaatcctgcccctagggttccaggctaaagggagaaagcgcaggaacctggcttcaaagggaggctggagtctgtagtgcaccacactgtctgcgtttgtgtttcctggaaaaccccagatgctttcttctcggcgatactgcttccagtttctcccaccatcactgaacatcaggaggtagctggtcacccagtcagagctcccatatcctccttgggtggcgacagcagtgacctccattctctctccaaggtcaatttgcagccattggtatttatttgacacaagtggagtccagccaccagctccatctcttcgattaagccttgaaaaccccgggccgtggctgctggacagctctgaggagctgctgaaggatgacctaggcaaggcagaggccagtggggcatcacagtcaggtggatttcctgctcccacggggctccaagtctgagtggggagaagcagcagcaccttgaggacggcccaggccactgaagccatgctcacttcagccaggcgccctgagacccgggcacggcgacggccgctctgcgtcgctcctgctctcactcccgtcccctgcgcggctctgacgctgctctgc

SEQ ID NO: 15717 - RNA, 1361 nt, Homo sapiens
  source 1..1361: mol_type = other RNA
gctgggattacaggcatgagccactgtgcccggcctgttatctttctgtatagatggggttttgctatgttgcccaggctggtctcaaactcctaggctctagtgatccacatgcctcagtctcccaaagtgctgggattacaagtatgagccactgtacccagccaacaaaacggttttaagtctgctttcttctcttttgtgggtgtggggagtcagcatttcttcaaactttgcacattataggtacttagtaaattatttactaagtgaatgatttgcttttctgcttgacacaagtagcttagtaataaatgtgcccaggcaaaatgccagagataccttgaagagctcagagtggtactccagtggaaaccagaccagttgttctgcccgcacttttaataatgatttggcttgcaaaactgatttggcaagagttttcaggaccactgttttattatcatactgtttttgcaacttgtaggcattgggctctgatgccattgccataaaagtaagtagccgtcgtaattcttctctaatgttcagcaacagcaatcttagatatagttgtgttgcttcaagtgcttctgctcttttctcattttctaaaagttcaataattcctgaatgaatatcaaaatactcatcagttaataggcaatctctctcttgagcatagtattttgctatgacatcaaagagtatcttcttctgactgttcaatcttgtctcttcatttctgttttgcattaactgctgactaactgtaactattaactggtcagggaaatactccaagcattcaattgctgcattaagccagttatcgatttcaggtagacataagcttggaataagttctctgtctaggcaagtgttagtgataacaagatcttcctctttgtttagttgaagattttgtgttttaactggaggctccaaaatattgtccaagaatggaaggtgaatcaattgaagaagacataataatgtttgttctttccaaacatctgtcttatctgatgtaattgctgtgtagaaggaaactccttcttttgaaagccggagaaaaggtttctgaactgtgatatttggacataaagctggattcccatttattgtatgaataagttcctcaattctttcctcaccaatctcctgtgctagaggatttgaaatcatttcatatcctggtctgtcctccttttccggcagaagccatctctacggttcctggaacttggcccgttcagccctgggcccggaagctcgttctgactgacaagtctacggaacctcggagtcaaaagaaccgccataagctcgcgcgctggctcctcccctggcaccatagc

SEQ ID NO: 15718 - RNA, 1719 nt, Homo sapiens
  source 1..1719: mol_type = other RNA
gctgggattacaggcatgagccactgtgcccggcctgttatctttctgtatagatggggttttgctatgttgcccaggctggtctcaaactcctaggctctagtgatccacatgcctcagtctcccaaagtgctgggattacaagtatgagccactgtacccagccaacaaaacggttttaagtctgctttcttctcttttgtgggtgtggggagtcagcatttcttcaaactttgcacattataggtacttagtaaattatttactaagtgaatgatttgcttttctgcttgacacaagtagcttagtaataaatgtgcccaggcaaaatgccagagataccttgaagagctcagagtggtactccagtggaaaccagaccagttgttctgcccgcacttttaataatgatttggcttgcaaaactgatttggcaagagttttcaggaccactgttttattatcatactgtttttgcaacttgtaggcattgggctctgatgccattgccataaaagtaagtagccgtcgtaattcttctctaatgttcagcaacagcaatcttagatatagttgtgttgcttcaagtgcttctgctcttttctcattttctaaaagttcaataattcctgaatgaatatcaaaatactcatcagttaataggcaatctctctcttgagcatagtattttgctatgacatcaaagagtatcttcttctgactgttcaatcttgtctcttcatttctgttttgcattaactgctgactaactgtaactattaactggtcagggaaatactccaagcattcaattgctgcattaagccagttatcgatttcaggtagacataagcttggaataagttctctgtctaggcaagtgttagtgataacaagatcttcctctttgtttagttgaagattttgtgttttaactggaggctccaaaatattgtccaagaatggaaggtgaatcaattgaagaagacataataatgtttgttctttccaaacatcttcttttgaaagccggagaaaaggtttctgaactgtgatatttggacataaagctggattcccatttattgtatgaataagttcctcaattctttcctcaccaatctcctgtgctagaggatttgaaatcatttcatatcctggtctcaaggtttcattgaactcattctcagcatccttttgtcttttgcaacaatcgtaagatgatttattgcctagaaacctgtagagactaatgttggaatcttcaaattctaattccttttcttttttgaaaagcttcttcattcctactggttcaaatactttgtgattcattagaacttggcaaagatgaacccctttaagacaagagatgtcattgctacttaggcacgtgttttgcataagatgacttaagaccacatcgacagcatcagaaccagtgaaacagtctttgtatgtctgtaaatgatgcctccttctttttatttccacttgggcctgaagagagtgaataataccatcccatagctgagtagcttgaaaaggaccagagcatcctgtcctccttttccggcagaagccatctctacggttcctggaacttggcccgttcagccctgggcccggaagctcgttctgactgacaagtctacggaacctcggagtcaaaagaaccgccataagctcgcgcgctggctcctcccctggcaccatagc

SEQ ID NO: 15719 - RNA, 1095 nt, Homo sapiens
  source 1..1095: mol_type = other RNA
gctgggattacaggcatgagccactgtgcccggcctgttatctttctgtatagatggggttttgctatgttgcccaggctggtctcaaactcctaggctctagtgatccacatgcctcagtctcccaaagtgctgggattacaagtatgagccactgtacccagccaacaaaacggttttaagtctgctttcttctcttttgtgggtgtggggagtcagcatttcttcaaactttgcacattataggtacttagtaaattatttactaagtgaatgatttgcttttctgcttgacacaagtagcttagtaataaatgtgcccaggcaaaatgccagagataccttgaagagctcagagtggtactccagtggaaaccagaccagttgttctgcccgcacttttaataatgatttggcttgcaaaactgatttggcaagagttttcaggaccactgttttattatcatactgtttttgcaacttgtaggcattgggctctgatgccattgccataaaagtaagtagccgtcgtaattcttctctaatgttcagcaacagcaatcttagatatagttgtgttgcttcaagtgcttctgctcttttctcatttttcaggtagacataagcttggaataagttctctgtctaggcaagtgttagtgataacaagatcttcctctttgtttagttgaagattttgtgttttaactggaggctccaaaatattgtccaagaatggaaggtgaatcaattgaagaagacataataatgtttgttctttccaaacatcttcttttgaaagccggagaaaaggtttctgaactgtgatatttggacataaagctggattcccatttattgtatgaataagttcctcaattctttcctcaccaatctcctgtgctagaggatttgaaatcatttcatatcctggtctgtcctccttttccggcagaagccatctctacggttcctggaacttggcccgttcagccctgggcccggaagctcgttctgactgacaagtctacggaacctcggagtcaaaagaaccgccataagctcgcgcgctggctcctcccctggcaccatagc

SEQ ID NO: 15720 - RNA, 2132 nt, Homo sapiens
  source 1..2132: mol_type = other RNA
gctgggattacaggcatgagccactgtgcccggcctgttttctttcttttaaaacaagaataatgaggcaaaatatttgagtgaaaacaaataacacaaaagcacaactcttggaggaaaaaatctgacatttaccaacagttttggggaggtgatacatcaacacttaaatgatgcaatccatcacgtgaatctgtaacgtgtctatgtcaggcagaacctctccacacttggggcaggaatgaatcggaatattccgctgttgccgccagtccctgtcctcagctcctctttgaacaaggtaagcctgctggtcagagtcacttgttctcgccccatgacgactctgcatctccatcaaggactgcctgcctccgtcttcgaaagcatcattctctttcagcagaactgccagctgcaatgccagttgctccttttcctcatgaattttctctctcgctgctctttcagcatgaaaatcagaacagtaaacttccatctgagccctgaggatggtcatggtttccaggtcctcttcctgcttggcaatggtttgcttcatttcatccatttgcagctgtttggaagccagagccttctctgccagttccagtttttcactcagttccttcagcactgccctgtccactttttctgactcttttcttgttagttcctcaattgttttcaatgcattattatgttcttgaagaagcttgttgtgtgtcatctgtagcacagttaatttggacttttcatcctctgttttagcctgttccattttgatttctgatagcatgctttccacttgtagctctaactttttgttagtataaacaagctcttgcttttcattcaactctgatggaattgcagaatttttcctttcaagggcctgacacttttcttgaagtctcttcttcattagctcagcttcgctgagttttgtatgagcctcttgaagctccttaaacagagatgtcacctggaggttcagtgcttccacttcgcttccaacagtctccgggcctttctcttcatcattctctttctctgtgctcccctctgtctgggtttcaatctcagaacgattacttgttttcttttcaaaatctgaaactctttctttggcctccttgagtgcaacttcaagtctctccaccttctgattcccttcccttaggcacagcaggagctggctcacagttaactcctcatgttcgaagtaattcttggccccatctgcagatctgctcctatatttagacaatgccgtgccagtggagactgttctcgtgggcccaggactatgcttgatttcttttactgacccttctgcttctccttcagccatcctaatttcaacaaaggaatcttctgaggagccgctggagttcagcttgagctgcagttcagacacgatgcccaacaggtctgccttctctgcttgtagcctcaccacctgggtcctgagctggtccttttcctgctccgcttcggccctgggaagcctggagtcatcagtggggtcctcagatgacctttctgatttcccttttagttttccaagctcttccttcaatttctcattctcatgactcaaggccattagacgctcttttgcttctttgctctgtatctcaaaaaactggcgttcttccttctgtttctctgtccaggccgaaagctcctcaaatctccctttcatggcttgattatttagcttcatggcttctttcagctggtggttctcggtcaggagctctttcatctgctgcagcagctcctccggggtaaacgtgtccaggtttgggtgggccaggtgggggggtccatttcctgtgctttcactggggctgtcctccttttcagtgaggcagctgagaggttgatgggacattgcagaagttcctgccgcccggcttggcttcgctcagggtcactgtttcctcggcatcgtgccgcctggagagaactcccgaccgggatgggacgctgaccagggaacctgccggcgggcggcggcggtggcggagggggcagccgggactggggtgcctagggctgatgcgcggcctggcgaccccgcccagcgcggctcagctgacagccagccgctccctgcccgcgcc

SEQ ID NO: 15721 - RNA, 2353 nt, Homo sapiens
  source 1..2353: mol_type = other RNA
gctgggattacaggcatgagccactgtgcccggcctgttttctttcttttaaaacaagaataatgaggcaaaatatttgagtgaaaacaaataacacaaaagcacaactcttggaggaaaaaatctgacatttaccaacagttttggggaggtgatacatcaacacttaaatgatgcaatccatcacgtgaatctgtaacgtgtctatgtcaggcagaacctctccacacttggggcaggaatgaatcggaatattccgctgttgccgccagtccctgtcctcagctcctctttgaacaaggtaagcctgctggtcagagtcacttgttctcgccccatgacgactctgcatctccatcaaggactgcctgcctccgtcttcgaaagcatcattctctttcagcagaactgccagctgcaatgccagttgctccttttcctcatgaattttctctctcgctgctctttcagcatgaaaatcagaacagtaaacttccatctgagccctgaggatggtcatggtttccaggtcctcttcctgcttggcaatggtttgcttcatttcatccatttgcagctgtttggaagccagagccttctctgccagttccagtttttcactcagttccttcagcactgccctgtccactttttctgactcttttcttgttagttcctcaattgttttcaatgcattattatgttcttgaagaagcttgttgtgtgtcatctgtagcacagttaatttggacttttcatcctctgttttagcctgttccattttgatttctgatagcatgctttccacttgtagctctaactttttgttagtataaacaagctcttgcttttcattcaactctgatggaattgcagaatttttcctttcaagggcctgacacttttcttgaagtctcttcttcattagctcagcttcgctgagttttgtatgagcctcttgaagctccttaaacagagatgtcacctggaggttcagtgcttccacttcgcttccaacagtctccgggcctttctcttcatcattctctttctctgtgctcccctctgtctgggtttcaatctcagaacgattacttgttttcttttcaaaatctgaaactctttctttggcctccttgagtgcaacttcaagtctctccaccttctgattcccttcccttaggcacagcaggagctggctcacagttaactcctcatgttcgaagtaattcttggccccatctgcagatctgctcctatatttagacaatgccgtgccagtggagactgttctcgtgggcccaggactatgcttgatttcttttactgacccttctgcttctccttcagccatcctaatttcaacaaaggaatcttctgaggagccgctggagttcagcttgagctgcagttcagacacgatgcccaacaggtctgccttctctgcttgtagcctcaccacctgggtcctgagctggtccttttcctgctccgcttcggccctgggaagcctggagtcatcagtggggtcctcagatgacctttctgatttcccttttagttttccaagctcttccttcaatttctcattctcatgactcaaggccattagacgctcttttgcttctttgctctgtatctcaaaaaactggcgttcttccttctgtttctctgtccaggccgaaagctcctcaaatctccctttcatggcttgattatttagcttcatggcttctttcagctggtggttctcggtcaggagctctttcatctgctgcagcagctcctccggggtaaacgtgtccaggtttgggtgggccaggtgggggggtccatttcctgtgctttcactggggctgtcctccttttcagtgaggcagctgagaggttgatgggacattgcagaagttcctgtggaaaagtcactccaaaagttgcccactttctctccagttacattttggacatttttgattcttctatgtgcggactcagcacaccaggcctgtcactgactaatcttcattaatgctgaaccaggcagctgtttcaaaggtgaggaagttgggtttacagaggcgtacggctcatccaaggccaggaagtggcaccaccagctatcaaagccacacctgccgcccggcttggcttcgctcagggtcactgtttcctcggcatcgtgccgcctggagagaactcccgaccgggatgggacgctgaccagggaacctgccggcgggcggcggcggtggcggagggggcagccgggactggggtgcctagggctgatgcgcggcctggcgaccccgcccagcgcggctcagctgacagccagccgctccctgcccgcgcc

SEQ ID NO: 15722 - RNA, 2203 nt, Homo sapiens
  source 1..2203: mol_type = other RNA
gctgggattacaggcatgagccactgtgcccggcctgttttctttcttttaaaacaagaataatgaggcaaaatatttgagtgaaaacaaataacacaaaagcacaactcttggaggaaaaaatctgacatttaccaacagttttggggaggtgatacatcaacacttaaatgatgcaatccatcacgtgaatctgtaacgtgtctatgtcaggcagaacctctccacacttggggcaggaatgaatcggaatattccgctgttgccgccagtccctgtcctcagctcctctttgaacaaggtaagcctgctggtcagagtcacttgttctcgccccatgacgactctgcatctccatcaaggactgcctgcctccgtcttcgaaagcatcattctctttcagcagaactgccagctgcaatgccagttgctccttttcctcatgaattttctctctcgctgctctttcagcatgaaaatcagaacagtaaacttccatctgagccctgaggatggtcatggtttccaggtcctcttcctgcttggcaatggtttgcttcatttcatccatttgcagctgtttggaagccagagccttctctgccagttccagtttttcactcagttccttcagcactgccctgtccactttttctgactcttttcttgttagttcctcaattgttttcaatgcattattatgttcttgaagaagcttgttgtgtgtcatctgtagcacagttaatttggacttttcatcctctgttttagcctgttccattttgatttctgatagcatgctttccacttgtagctctaactttttgttagtataaacaagctcttgcttttcattcaactctgatggaattgcagaatttttcctttcaagggcctgacacttttcttgaagtctcttcttcattagctcagcttcgctgagttttgtatgagcctcttgaagctccttaaacagagatgtcacctggaggttcagtgcttccacttcgcttccaacagtctccgggcctttctcttcatcattctctttctctgtgctcccctctgtctgggtttcaatctcagaacgattacttgttttcttttcaaaatctgaaactctttctttggcctccttgagtgcaacttcaagtctctccaccttctgattcccttcccttaggcacagcaggagctggctcacagttaactcctcatgttcgaagtaattcttggccccatctgcagatctgctcctatatttagacaatgccgtgccagtggagactgttctcgtgggcccaggactatgcttgatttcttttactgacccttctgcttctccttcagccatcctaatttcaacaaaggaatcttctgaggagccgctggagttcagcttgagctgcagttcagacacgatgcccaacaggtctgccttctctgcttgtagcctcaccacctgggtcctgagctggtccttttcctgctccgcttcggccctgggaagcctggagtcatcagtggggtcctcagatgacctttctgatttcccttttagttttccaagctcttccttcaatttctcattctcatgactcaaggccattagacgctcttttgcttctttgctctgtatctcaaaaaactggcgttcttccttctgtttctctgtccaggccgaaagctcctcaaatctccctttcatggcttgattatttagcttcatggcttctttcagctggtggttctcggtcaggagctctttcatctgctgcagcagctcctccggggtaaacgtgtccaggtttgggtgggccaggtgggggggtccatttcctgtgctttcactggggctgtcctccttttcagtgaggcagctgagaggttgatgggacattgcagaagttctatgtgcggactcagcacaccaggcctgtcactgactaatcttcattaatgctgaaccaggcagctgtttcaaaggtgaggaagttgggtttacagaggcgtacggctcatccaaggccaggaagtggcaccaccagctatcaaagccacacctgccgcccggcttggcttcgctcagggtcactgtttcctcggcatcgtgccgcctggagagaactcccgaccgggatgggacgctgaccagggaacctgccggcgggcggcggcggtggcggagggggcagccgggact

SEQ ID NO: 15723 - RNA, 2338 nt, Homo sapiens
  source 1..2338: mol_type = other RNA
gctgggattacaggcatgagccactgtgcccggcctgttttctttcttttaaaacaagaataatgaggcaaaatatttgagtgaaaacaaataacacaaaagcacaactcttggaggaaaaaatctgacatttaccaacagttttggggaggtgatacatcaacacttaaatgatgcaatccatcacgtgaatctgtaacgtgtctatgtcaggcagaacctctccacacttggggcaggaatgaatcggaatattccgctgttgccgccagtccctgtcctcagctcctctttgaacaaggtaagcctgctggtcagagtcacttgttctcgccccatgacgactctgcatctccatcaaggactgcctgcctccgtcttcgaaagcatcattctctttcagcagaactgccagctgcaatgccagttgctccttttcctcatgaattttctctctcgctgctctttcagcatgaaaatcagaacagtaaacttccatctgagccctgaggatggtcatggtttccaggtcctcttcctgcttggcaatggtttgcttcatttcatccatttgcagctgtttggaagccagagccttctctgccagttccagtttttcactcagttccttcagcactgccctgtccactttttctgactcttttcttgttagttcctcaattgttttcaatgcattattatgttcttgaagaagcttgttgtgtgtcatctgtagcacagttaatttggacttttcatcctctgttttagcctgttccattttgatttctgatagcatgctttccacttgtagctctaactttttgttagtataaacaagctcttgcttttcattcaactctgatggaattgcagaatttttcctttcaagggcctgacacttttcttgaagtctcttcttcattagctcagcttcgctgagttttgtatgagcctcttgaagctccttaaacagagatgtcacctggaggttcagtgcttccacttcgcttccaacagtctccgggcctttctcttcatcattctctttctctgtgctcccctctgtctgggtttcaatctcagaacgattacttgttttcttttcaaaatctgaaactctttctttggcctccttgagtgcaacttcaagtctctccaccttctgattcccttcccttaggcacagcaggagctggctcacagttaactcctcatgttcgaagtaattcttggccccatctgcagatctgctcctatatttagacaatgccgtgccagtggagactgttctcgtgggcccaggactatgcttgatttcttttactgacccttctgcttctccttcagccatcctaatttcaacaaaggaatcttctgaggagccgctggagttcagcttgagctgcagttcagacacgatgcccaacaggtctgccttctctgcttgtagcctcaccacctgggtcctgagctggtccttttcctgctccgcttcggccctgggaagcctggagtcatcagtggggtcctcagatgacctttctgatttcccttttagttttccaagctcttccttcaatttctcattctcatgactcaaggccattagacgctcttttgcttctttgctctgtatctcaaaaaactggcgttcttccttctgtttctctgtccaggccgaaagctcctcaaatctccctttcatggcttgattatttagcttcatggcttctttcagctggtggttctcggtcaggagctctttcatctgctgcagcagctcctccggggtaaacgtgtccaggtttgggtgggccaggtgggggggtccatttcctgtgctttcactggggctgtcctccttttcagtgaggcagctgagaggttgatgggacattgcagaagttctccaaaagttgcccactttctctccagttacattttggacatttttgattcttctatgtgcggactcagcacaccaggcctgtcactgactaatcttcattaatgctgaaccaggcagctgtttcaaaggtgaggaagttgggtttacagaggcgtacggctcatccaaggccaggaagtggcaccaccagctatcaaagccacacctgccgcccggcttggcttcgctcagggtcactgtttcctcggcatcgtgccgcctggagagaactcccgaccgggatgggacgctgaccagggaacctgccggcgggcggcggcggtggcggagggggcagccgggactggggtgcctagggctgatgcgcggcctggcgaccccgcccagcgcggctcagctgacagccagccgctccctgcccgcgcc

SEQ ID NO: 15724 - RNA, 2947 nt, Homo sapiens
  source 1..2947: mol_type = other RNA
gctgggattacaggcatgagccactgtgccctgattattttttattttttttgagacagagtcttgctctgtcgcccaggctggaatgcagtggcacgatcttggctcactgtaacctctgcctctcaggtttaagtgattctcatgcctcagcctcccaagtagctgggattacaggcacctgccaccacgcctggctaatttttgtatttttagtagagatgaggtttcaccatgttggccaggctgttctcaaactcctcacctcaggtgatccgcctgcctcggcctcccaaagtctgggattacaggcgtgagccatcgtgcctggcccagccttttcttaaatacttccagagacagggagctcagtgcttctagagtccatctgaccagtgatccgcatttggaccacattagaaaagtctgtcttctttttcctagggaaatttgcctcccgaacaagaacccgctggtccaagctttgaatgcaggtggctgcggccagcgcactggatttatcttcccgaatgacttctgaaacactcaaacgcccgataccctgtatcttcctcttgctaggtctgcctatttcagagccagtttctgagcctctgctgttccaacccggaacagcgttggcgtgtcccagcctgacgctgggttgggggagcagtgaggtccacatatctcattccttggtgggaggtattgacggggtttgcccggtggcttgacatctgagttaaaggggcttgagaatgttctagattactggggtgtcattttgcaatcggaggacaaggatggttggcagcggctcttcttgtgcaatgggctctgatcctctcaaaggagctgggtgtcattatgagcgagaagggggcgggtcaaatgaaaaaccatgggtgtgaaatttggacataaggtcggaggtcaggagctaccccaggacgtggccctcataggggggttgagcttctaggtctgaggccgcattctggagggaaaggcacaggaaaggacgcagacccagccggggtggcggtgggtgtctgtggctccaacctggagcgggtgacaagcaagagaagggtcttgaatcttgtatccagctctgaccacagaggctgcgagcaggagcggaggccaccgacgccacgcgggccaccccctgcgcttcttgccttcctcggctgagagttcgtgagtgtggaagggtgaggggctcagagctgggcccttttctggaacgcacaaatactgcatcgttaaaaaaaaaaaatacaatgttttcaagcagctgaaaaggatgctgggtttcagagatgaacggaggggctggcacccttggaagattgggactcaggatgaggcaggatgagatctggggccagtgggcgtctgacagaggttttctggcatctggaatcttcttccatgtcctttgttatgctcacgtcgcctcaggacatgcttgtttcctgatcttctgagaccagagcagacctgttttccactggtgccacctctggcttctcttcagacctgggcagcacaaactccggctggggcctcgcgctctccctcctggccttcagtctttcctcttcgtattgcaggacgcagtctgggatctggacgtgttccatagggatgagttgctccaggtcttccaagctgtgcacgtactggatcttgttgatgaacttgacgctgatgaaagggcgagagatggccagcacagtccgaatgaaccacgaggggtggacgatgatcaaggacttcaggtttttccgcaacctccggtcgatcatctggtagcacttcttcagccagccgattccaggcatcctccgccggggcgtggcaccgttcaggtacacgatcatgtagtcctcagccaccaggagctctaagctgctgatgacgtacaggaagaggttctccatgatgtagtggtagtcggggaggctgctgtctggaaggaagcaggctgcgaagacgatgatggcgttgaggccttcgccgtagtaccctccgtgggtgaccactttcatgtaaggccggatcatgtgcaggtctatacggtgctcttgctccccgatgatcactgtccgccacaggcgcccgttggcggcgctgccgtcctccgtcgtgccgtccccaaatagatccgcgctgtccccgggcatgttcttggcggtggccacgggggtgtcgtcttcccactccagttcgttgccattccccaggaactccagcgagtcggtctcatcgggggtctcgatgtcatccacgttaatatccaggtcatcaggggtatccaagaagtcatcggacagcagggacccctcactctgatccagagaaatgttgatctctggggccaccagcgtcttcctcttacgatgcgctccgttgaaatttagcgtgttgggaggagaggatgtgtcttccaccgggctgccaagcagttccacccccgtctcttctgggagtggcctgggaagatcttcgtcctgccattcctccttcacgtccacgttttccatccggagcgtggcttcggtggtccccatgggagctgggaagaggcactggcttgaagcagggatgacccctctgcagctgagacagcctctcctccttactggcaaacaaaggcgagccctgcccgggtgcagctgggcatcgctcacgctccccgggccttcagagcctaggaggaagaggatgctcgcaggggcggattctgcatccgaggaaggtcacccagggcgacgtggccagcgcccgccagctcttttgtgcaggggtgggtggggtgcagggttagcggtgggctccccagcgcggggctgcggctgcgccccctctcatcgccgcccgcctgcgcgccctgcctccgaggtagctgcttcttcccagctcagggctggcagag

SEQ ID NO: 15725 - RNA, 1435 nt, Homo sapiens
  source 1..1435: mol_type = other RNA
gctgggattacaggcatgagccactgtgcccttcctacatttctgtttttattctaccaataattttaaagtcagcttgtttagcaaagttatacttaagtcaggtgaacttgaaaattgcttaaacttatttactttatttatgagtgctcttttacttgtaagccaatttggtagacacaatgtattacaataggtgtacatacaaataaacacatctagacatgtagacccacacataaacgaagaaccaacagcttggaaccttagctgtgagatagcaatacaagcttgttggcatttactttgtctcaatagataatccaacaaaggctgtgaaccaaaatttcaggtaaagcagtctccatggagcttgatttttcaagaccaaacctctccagattccaaagaacactggggccaaacagcacccaaggagcatgtcacatgttaaccaggccccctgcttagaacagcagcaacaaaggctggatacatgcaatgccatcccactttcccattcaacaggaaactccagattccaaactatactggggctaaacagtattgcaaaccggagagaaaattctaaggggggcttagtactagacctcaaaacctctgccgagagcaccccctttggagaggttgagattcggaggatcctcagggcgtccccctatggggtccaaaagagtgtcagacgtctctgacctttctctgcatgttttccctccagagcctcctatgagctatgagcttgataaggatagccctgaactgtaatgatacataggaactggatgctgggtgggcttttttgtccttagatagttgaataggacaagcaaaaaacttagcataagaaaaggtttaagtcacctgaaacaagtgtgagttaccaccaccaccgtagggatcagggaccacacctggaaaagataaaaaaaaaaaagagtcattcccccttctgggtagggcaattattcccattcactctttggccttcaggcgataccagggagtgaccccagcgaattgccctcaatttccaagaagctactaggaaacagccgctaaaagactgaaaaacaaacaaaggaaaagaaaaaagaaaaacactcaggtcccttaagtgaatagggtggtggtggttaggcacctccacatggaaaccccttatttcactggtcacagccagaaacctgcagttgcttccatgtttctgcgcttcccaccaagggtcccgaggtggaaaggaacagacagacagagaaaaatctccctgtatgtaaaaggggaaaggagaaaaataaatcccaaactttgggcctaccttctcctggctggctcgccaaaatatgttaccggtggagggtgtccagtttcttggtgtctgtagttccagctactggagaagctgaggcaggagaat

SEQ ID NO: 15726 - RNA, 1096 nt, Homo sapiens
  source 1..1096: mol_type = other RNA
gctgggattacaggcatgagccactgtgcccttcctacatttctgtttttattctaccaataattttaaagtcagcttgtttagcaaagttatacttaagtcaggtgaacttgaaaattgcttaaacttatttactttatttatgagtgctcttttacttgtaagccaatttggtagacacaatgtattacaataggtgtacatacaaataaacacatctagacatgtagacccacacataaacgaagaaccaacagcttggaaccttagctgtgagatagcaatacaagcttgttggcatttactttgtctcaatagataatccaacaaaggctgtgaaccaaaatttcaggtaaagcagtctccatggagcttgatttttcaagaccaaacctctccagattccaaagaacactggggccaaacagcacccaaggagcatgtcacatgttaaccaggccccctgcttagaacagcagcaacaaaggctggatacatgcaatgccatcccactttcccattcaacaggaaactccagattccaaactatactggggctaaacagtattgcaaaccggagagaaaattctaaggggggcttagtactagacctcaaaacctctgccgagagcaccccctttggagaggttgagattcggaggatcctcagggcgtccccctatggggtccaaaagagtgtcagacgtctctgacctttctctgcatgttttccctccagagcctcctatgagctatgagcttgataaggatagccctgaactgtaatgatacataggaactggatgctgggtgggcttttttgtccttagatagttgaataggacaagcaaaaaacttagcataagaaaaggtttaagtcacctgaaacaagtgtgagttaccaccaccaccgtagggatcagggaccacaccttctcctggctggctcgccaaaatatgttaccggtggagggtgtccagtttcttggtgtcttgaacaaagaattagacaaaaggcacaaacaaaataaggaaggaatgaagggatttattgaaaatcaaagtacacagctgggcgcagtggctcaagcctgta

SEQ ID NO: 15727 - RNA, 1668 nt, Homo sapiens
  source 1..1668: mol_type = other RNA
gctgggattacaggcatgagccactgtgccgggccacattcctctaatttctaatatagtcaatgtcatcaaatacatcaacatcttgggggttctcacgagtggtcaaagtgtcaaagcgtcctgggccctcaatctctgagaactgtgggtccatagcccctgaaggaagtcagtggtggctctctgcatcctgtgttaaatttagcacttgctctcatgtatgtataacattttccccaactacttgactctccggggcagggcccacatctgactccatcgtgtgtccagcacagaaaaggacaggtttcgagctccctgtcaagggcccaagaacgagcagcagagagaatgtctgctgtcgcctgcacatcgacgtcatgatgtcttcctcctgtcacagctgcgaccgagcggctcagggagttgggcaggccccagctgctcccagaagctggtcacagcttcgacaggtactgtcttctggtaggcagaggacacctgggtgacatcctcaaaggttgacgcattcttatccatccgatccttctgcaccccatacttcccgccgaatcctttggagtagtcttgctgggactcgtgcttggccagcttctccttgtaatcaaaccccacagcagcggagtcctgcctctccgactgaacaccgaatttgcctccaaaaccagtcttataatctttttgggattcatgcagctgcaatttctcctggtgatcccagccaagggcacatttgtcttgtctgtctgtctgcacaccaaattttcctccaaaccctttcacatagtctttctgggactcgtgcttctccgttttgccttgatactcaaagccaacggcgctcttatccactttgtccttgtcgataccgtatttgccgccgaaacctttggagtaatctctctgtgactcgtgcttctccgtcttgccctggtagtcgaagcccaccgcgctcttgtctactcggtcggcctgcacgccatacttgccgccaaaaccactggagtagtctttctgggaggcatgcttctcagtcttcccctggtattcaaagcctacagcagactgatcaactctgtccatctggacaccaaacttgcctccgaagccacggaccgagtccacctgcgagcagtgcttggaaagtttcgactgatattcgtggccgacagctgacttatccattcggtcttgttccacaccaaatttccctccatagccatgggaagcttttggtcctgtttcaagttccttctccttaagggtctgatgctcttgaaagacattctccctcagcttgtgtatgttgatatgctcctggtgcccggagccctgcaccgtcttggcaccccatctttgctccttctcactcacatcattcacaaaatcagggtcggtctcccagtcatcggcccccgcgtcatcctgggcgatggacacagcgtggcctgctgaagctttccacatctttctttccgcttggagataaaaggctgttcacgaaattctgtttaaaacacagtaatccaatgaggaatttccaggcattggggactgattccgtcgccgcctggggtcggtccggcccgggtcggccctggattccgccgcgccagccgctcccaggcaccaggctctacttcc

SEQ ID NO: 15728 - RNA, 1116 nt, Homo sapiens
  source 1..1116: mol_type = other RNA
gctgggattacaggcatgagccactgtgcctagccaacatgggacatttctaactcgagggtattgtcaggccatgtaggaaagggagcagagattgcccttgaggagatgctcccaggtggcagatttgtcctacttgatagattccaaaatggaaaacggatttttctgctgcctctggggacactgaaaaaagaacctccacatgagttcagaggcagcaccggcagcttaggggaagtcatggcttccactgcgtgtctaggaagcgctctttcaggatgctctgaggctgccactggcacaggggaatactgtgcttctcatcagactgggctgcgggctgatgtgctcttgggagatgagctctgctcaggagcaagaggttgtgaaagggctgatgtttcttaggctcccccaatgagcagctccaagcagtgctgagatgtctaggccgtttgtgtcacaggacaagcacacttgcagacccaactgttggaatccttcattggcatatcattcccattgctgctgtttgtctccacatcagaattgcttgctatacttagccagaagccctgccacattgcagtgcagaggcttagctttcttgtttttgttgctgagtgctctgagataccagtttgtccctttgtggtgatttaggcagttaggtggcctttgatctcattcacagagtaaaaatggctcaggaggagccagcagacactagcgtacacatttccaaatgtcatctttctagagccttctctttggggttgtcacctctcctatagaatttggtagaatcacaaagtggtctccaagagagtgtgaataggaagtaagagtgagcaggcaggccatgtaattggaagtggaatatctctgctctcaattgataattaggaatcttcttagatcagccttacaggtgaagaattgtggcacctgctcaggagcacatcctcggcattgcctcccctcccttccatgaggtcccatttcttgaggttgatggagacaggactaaaacccaggtcttccctttaaccaacctccacgtgcgtgttaaccgcggtgacagcatttccttgtctctctgctcccgccccc

SEQ ID NO: 15729 - RNA, 2010 nt, Homo sapiens
  source 1..2010: mol_type = other RNA
gctgggattacaggcatgagccactgtgcctagtcaatattttcaatttgtgatgtgtttacatcctgataaacccattgtaagttgaggagtatctgtacctgaagatagcatcagatcccacagagtgaaggctcagtcccacaagactctcccacttccaatgccaacacaagcttcaggttgttttatctgtgcctctgaccaaccagctataaatcgaggttctcaggactgctccttgggttcaattaatttgttagagtagctcacagaactcaaggagacacttacttacgttcatccatttgttataaaggatattttaaaggatacaaataaacagccagatgaagagataccgaggggaagctctagaagggtccggcgcataggagttgctgccctgtggcgttgggtttgcaccctcctggcctgtggatgtgttcttgttcaccttcctggaagcccccaaactcagtccttttggatttttatggaggcttcattacacaggcatgaccgattaaatcattggcaattggtgctctactcaatcttcatcccctctcccttccccagaggtgaggggtgggcctgtaaattccaaccctcagagcaccaggtttgttcccctggcaaccagccccccatccagtggctatctgggactttccaaaaatcgcctctttaacataagctcaggtttggttgaaaggcacttgttcctccttagtacagtggttagtaaaattaactaattaaaataaaatgaaagattaaactaaaagaaacgggcttgttataaataacaaaagactgtctttcacctttatcactctggagctgttctggagctgtttcagaaaccaaggacaaaaggtcaaatattttaacaaaacatactattattgctctagtcccttaggaaattacatgggttataagagctgtaagccaggaacatatcgcacccagcatggggagagatggagaggcagtctccaaggatctgggggagagacttcggcttggttcattctccattcccaaaacgccaatgtctcaaagcttcctcttatgcatccaggctgaggctccttgggaaggtttggagctggagaagcagctgaatgactcatgcctaaggggccggtgccattcagatttatgacttccttgagaacaaagattatatcttattcacctcaatatcccacatctgatgctccataaacgggttttgaattgaattgctcccctcatattacctatccaggccacctcctgacctgtccccagcactcttcggcctccctgcccattccttcccccactccataacttcacctccaaactgtcacttccatctgcttctcggtctatgatgtcaaagatgtcttcatgaattttctcaccctctggatgggaatatcaaaggtctctggaatggtcgctaggacacctgggagaatccgctggcccagttgttgccagctcctcctccatgttccgacaggtagatgttctctgggttgtagagcttggcatagggggagttgaggatggagtggatcacccggggttccaagtccagcagcacggcccgggggatgtagtgctcatcgtctgcctggtagaaaaagacgtccttgcggtcagtgccctcggtggcgaattcctccacgatgccctcggggctgataccatgctcggcgcacagctgtttccagaactcgaacccaatctggttgccgcactggcccagctgcagggtgatgatctcccggggcatcgctcttcagacgtgggcgcgccagccccggcctggcgagagtcacggctgagacgaatgcccggcagccaggagcgcaggacgtggggagcgcgcgctctcttcgcctcttgacgcggatgctcggtctgcgcgtgtgcagcgcaggcctctcctcggccggtgggccggggagcccaacctgggcatcattttctccctcagcagtcgcagct

SEQ ID NO: 15730 - RNA, 1879 nt, Homo sapiens
  source 1..1879: mol_type = other RNA
gctgggattacaggcatgagccactgtgcctgcatgtcttggttttataggggagaaaaagaagtctgctgtgtcctgctaaatccccttgtgggtgacattgcccttctcagctacataaataacactggaaagagaaccaggtgtgcacagcacaaggctgagcaatttttctagaatactcagtcccaggctaccctttaccacatccaacaccacagtactgcaagggcctgacagggcgcctctcttcggctctaagatgggcttgagagacagggcatggagggctgcctgcatgggggcccccaatcccagaatttcattcatgaactcaagaggcctgtttccgcagcacgcggcagctcatacatacaaagctgcaacacgtggtcaccacgtcctgatgtccactgtgtgaacaacacaaggggagctccaatctgcatctctgacctcctggttagagggtggctgatcagatctgaaggccctcaaagtgaaccattcactcacctccatcagctccaggaacaatctaagacatcaagatatgtgtcatcagcaacgaaccacagtggtaaccactctccatcctccttcctgtgccagtcgggcggggacctccacctggactccgggagccaccatctgggcagcctgagctgtctgtactgctgtctgctgctgctgcacctggggctgcactgggggctgctgcaccaccatcggagctcggacaaatttcagtggtggttgggtatacaacatttgtccagggagagcttgcgcctgtgacaccaaaggctgggtctgcgactgtggcgggagttgtgatggttggttctgagcaactggaggctgctggggctgtggtggcggctggtggtgctgtgtgtgatgcatctgctgcagctgctggggcagagcctgggagggcggaggctgtggctgctgcatcggtggctgctgaattggtggctgggcctgcaaagcctgctgctgctgctgctgctgctgctgctgctgctgttgctgttgttggagctgcagctgtgctattcgctgcagctgctgttgctgctgctgtatctgttgctgattttgatgatgcaatttaattagatgctgctgctgctgctgctgctgctggagctgctgctgctgctgcactactgcttggaactgctgctgcatggcactctgctgagcctggaactgctgctgttgctgctgctgctgctgctgctgtagcgccgcctgctgctgctgctggaactgctgctgttgctgctgctgctgcagcgccacctgctggagctgcagctgggtctgtggagttgccgtagacacgacagccatgctgtgaggggccatccccgaggtcccaggaggcggctgccctgagagagacattggctgtcccatggcaccaaggctacccatcccgcccagagactgtcccgggccccgaggaggcatgccaattccagcggctcccgcagcaggtccgccagtcaggctctggagtgcattcataggatcactgacggaagcttgagatttcttgttatgaatgtctcgaaaatggataatgagcctggccacgagagaaaggtattcgtcccgggtcttggccttcaggaaaacatggctctccatatccttgctggatttactgtgtgccacaccagctttcctcatggcatcctcgatttgactgaccagcttctgccggaaggcggtgctccgccagtcggtctcttgcccggaaacgtccatgcctgttccccagctcccgccgcccgtatcccgcttggccgccaccgccgccgcctcagtcacagagccaggcccaaacccggaagccgtccgcagt

SEQ ID NO: 15731 - RNA, 5136 nt, Homo sapiens
  source 1..5136: mol_type = other RNA
gctgggattacaggcatgagccactgtgcctggcaagcaaatcccatctttttcacctctctgtctggcttatttctactcatcctttgggtttaggtatcactttttcaaggaagcatttcaggagccctccagtgtgtctcatgctctaacagtgagtgcaaagaacctccattcttcctctagcacagcttgaaatgaccagactccttctctataatttccactgggcaataagttccctgagggaaggaagcttctctgtctttagttgcatatgctctgtgactggcacagggtagatactcaataagtgaataaacagaggtctctcaagcacattcccttggtaagaaataccacccaagcagaaagagagacaataggaatttttaatgcatggacaggcctgcagggactctgggcagacccacaggtagcaggaagaggcagggtcccacaaactcaataatgtccagcaaaaaagagagagaagtccttaaagacccatgcttcctcactgcaaccatcctcagagcttccttcctggtgctgaagaggtcaaaactgtctcctctaggggtcaggtcaaaactgtccctccataggtctcctccaggggtccatggcaggaagaaagcagagtgtggcaggaagaaggaagaagagcaaaggccgcttggtctccacctgaaaacttctgcctcgggattgacagccatccataagaaaaggtttaaaaaggagagacttttgatagagtcaaataatatctttgaaaaaataaaagatagagaaaaatgaataattccattggttacaaaggtctctgtccactatccacaggagaaaccgtttgctttggccttgctggcaagcttcatctgctaggcccatcctcagctgtcccccagcccacccaggccccaggatccaggagaatactgctccccctcccatggagagtctctgtgctcacggagggcaataccctccctcaccggcccttggactccccgtacgtgtttcgggccattgacaccatcttctcctcacacgtgattttggtgtccttgaggatgctataccacaccatgcctgcaggccggacctcctcgctgcggcagaaaagatagggcactgtttccacgcggctctggatgtaggcactccgcaggaggctggagcagtggctactcaccctctccagtcgccgtagaatcaggtgggccttcctgggccccagctcatcctcacttctccagacgaagtcgccaaacttttcatagtgagagttgtagtggtgctggactcggaacagcatcgaggctgagacctccatcagtgtgttgtaggccatctgctgctcctttccacttgtgtacccattgtacagattgtagatcttgtcagctatttcttctgccttgttgtcatctaccagtggacaggccgtcctcagggtcaccgtgcttagctctgagtgcctccctcgtgtatccacagcatacagagtgaacttgtagagaccgtcgggctccagacacttgaagatgactgagtagatactgacttcagggacctctccatggcttcgaccagctgctacacaagatgtgcccaggccagagagtaagtcatcagcaaaactcaggaattctcctgtgtacaggtcagtgtctgtgtattcatccactttcttatgctgcagaatatagtcggagaccttggtcccaatagctggctgaacatccacccactccaaggagaccacagtactggagggctccactgttggggacagccgcagcaccggctgcagaagggggctgcagttggggagcccattggcatcaaaggcgctgaggtcacacctgcaccagtcatcgatcacatcccctttccctgagcaccagtaggaactcatcagtgcactcttgaaggcctcctttgtgccattgtcttggatgagggtataaagtggcaccacacggttgatttccagcagcactggtgtggggctcagctgctccttgcctggccggcggcaaaggtgacaggtagatggacagcgccccttctcctcacagcgaatctccacacctgaaatgagctggtcatctgacagcatctgggctgtcagcaaacctgagaggtaggtgatgaagggcatggacttgagctccttcttgctgcccagctctgtggtctctttctgatactggagccacagctgctgctggaccttcttgctgggaaagtggatgatgcaggtgagctctgagccatagagggcctctgcgatgtagtgggagccatagtgctggatgaaggacagcagctcctcccgactgctctccttggtcaggatcttgagaacattagtgaagcctgctgcgagggtgatggtgctgagcttcacacggtagaggttgctccggacccgccactgctgcaccatggggtaacccatggcctcatcatacctgatatctccagtgagcagttggaggtctggaaggggctcggagaggaccccccggcactgctcctccaccggcagcgggatcaccaacagcccatcggccagctggggaaagtccttgatgaagttgttctccctaaaggtcatctggaagacttggccttggttcacatgctgggtccggttgttgtaaccatgtagcatctctccaaagagggtatcattgaatttggagtcaggtttgaggcacttggggccctcgcagacatctgagagcattaagcaggattttccatcaggagccagtttgtactcctccacgcaaccgcagaacatgaagatggtgctcgaagtggcatcgtagggcaggggcagcgtctgctgcaggcacagctgctcacagccgccattaaagccatcagagcagtcaatgcctttggagtggtcgtagcagccagagccatccttcatgggtttcagctcctcagggcacacacatcccgaggaatccacctgccggtcagacacacacttgaagttgcgagtgcagcccccattgttccgagagcagtcacgaactggcccgaaggaagacagcaggtcattgatggtttcaaagtatgtggacagcatcgcttcttccctgacatctgcagggtcttccgtgacgagcacatcggtcttgcagctggccagggggttgatggacagctccacaggcggaaccacaaagcttttgctgacaggaagccagaggccttggcccaagctgaaagtagacctgagaatcttttcaggggcttgctcccctgtcaccagatcatagcccctctcaagtgtcgtgtagggccaaggtccttcactctgtccccagtcactgcgcacacacaggtgtctgtgaacagggtcaggggcatagccttcatgacagctgcactctccggtttctgggtcgcagagctgctcacaggcatctgtcgtcctttgtccacagaggtccctcacccatggggaggtggcattgatctggtaatacagggaaagcttggccgggtttaaccagtcggagatgtccaggtagctcccttcactcaccacgaagctgcttccatctgctatgaagtgctcgggcacatgcagagtcaccttcacagtgagtggacaagacatctggctgccacacaccatggccaggatgcaggaactcacagcaatcagtgtcagggctgtcttgttcactgggcttttcagcaaacctttgctgcggcggcgactgcggtactgctccgtgtagaatgtcagctgagtttcatcgtctgcctctgagcccgacgtccccttggctctcccaaagctgattcctcctcgagacttgctcctccgcttcctcttccctgccgatgtgctgcgcaggggtggttgcagctgaccgatctcgatgggcgtgttagcgcggaaactctccttgaacttctgcatcagggactccactgtctcctgagtcgcctcagctgctgctttcttctcaaagtccaccttctcttcccctggatgtcccagactgtccagagtgtgggtcacctggctgccaaactcgtcctcgcgggagacatggttggcccgcctaggtggctcctcatcctcctcacagtcatagtcatccaggatgggagtctcccggatgggcacgccaatgacggaattgtgggtttgcagccgggatgaacggaagctctcccgcgcctggggacccagcagcacagatgggatgtagtggatctcatgagtggcttctgtgcttgcgctcttctgggggatgcggcgacgcttctgccaacgtcgctgggcgtacagcgccacggtgaacaccagcagcagcagcagcagcgcgatgaggccacccatcacagaaatgtggaggatgtgcatctgctcctcaacaatctccgagggctcctggagagtgggggcggtggcttgggccagctgcccggagctgctcatggagacgtggaagtacaaggtgccattctccagccactgctgtctccagtgcaccagcgagatgtccgctgctgtgccagacatctccagggtgaagaagggcagctcggtgttgtccaggtcgtcctgcaccgcgatgcgccccggcagctcgttacgcacaaagagcaggaggcgcgactcggcggcggtgccggcagagccaggagagcccggggacgcggcggcggcggcggctccggccccggtcccagccccggccccggcgcgggcgccgctccagccgatgtcgctctcccgcagggcgggcagtgtggacaccgtgacggtcttcagccggcacgggctgtcgggctcccgcgaggcagcggcggtggcgccggccagcagcggcggcggcggcagcaggagcaggaacagcagcagcagcggcagcagtggcggcggccccgggtggaagcagagcctcggccgcccccggagccccgagccggggccggggctgagccgggcgccggcggcggccatggcgggaggggctgcggtgctgcgggcggcggcggcggtggcggcggtggcgaaggaggaagaggaggcagctgcggagacggcggacgccgaagcgaaccaggacgcccgagctaagg

SEQ ID NO: 15732 - RNA, 4983 nt, Homo sapiens
  source 1..4983: mol_type = other RNA
gctgggattacaggcatgagccactgtgcctggcaagcaaatcccatctttttcacctctctgtctggcttatttctactcatcctttgggtttaggtatcactttttcaaggaagcatttcaggagccctccagtgtgtctcatgctctaacagtgagtgcaaagaacctccattcttcctctagcacagcttgaaatgaccagactccttctctataatttccactgggcaataagttccctgagggaaggaagcttctctgtctttagttgcatatgctctgtgactggcacagggtagatactcaataagtgaataaacagaggtctctcaagcacattcccttggtaagaaataccacccaagcagaaagagagacaataggaatttttaatgcatggacaggcctgcagggactctgggcagacccacaggtagcaggaagaggcagggtcccacaaactcaataatgtccagcaaaaaagagagagaagtccttaaagacccatgcttcctcactgcaaccatcctcagagcttccttcctggtgctgaagaggtcaaaactgtctcctctaggggtcaggtcaaaactgtccctccataggtctcctccaggggtccatggcaggaagaaagcagagtgtggcaggaagaaggaagaagagcaaaggccgcttggtctccacctgaaaacttctgcctcgggattgacagccatccataagaaaaggtttaaaaaggagagacttttgatagagtcaaataatatctttgaaaaaataaaagatagagaaaaatgaataattccattggttacaaaggtctctgtccactatccacaggagaaaccgtttgctttggccttgctggcaagcttcatctgctaggcccatcctcagctgtcccccagcccacccaggccccaggatccaggagaatactgctccccctcccatggagagtctctgtgctcacggagggcaataccctccctcaccggcccttggactccccgtacgtgtttcgggccattgacaccatcttctcctcacacgtgattttggtgtccttgaggatgctataccacaccatgcctgcaggccggacctcctcgctgcggcagaaaagatagggcactgtttccacgcggctctggatgtaggcactccgcaggaggctggagcagtggctactcaccctctccagtcgccgtagaatcaggtgggccttcctgggccccagctcatcctcacttctccagacgaagtcgccaaacttttcatagtgagagttgtagtggtgctggactcggaacagcatcgaggctgagacctccatcagtgtgttgtaggccatctgctgctcctttccacttgtgtacccattgtacagattgtagatcttgtcagctatttcttctgccttgttgtcatctaccagtggacaggccgtcctcagggtcaccgtgcttagctctgagtgcctccctcgtgtatccacagcatacagagtgaacttgtagagaccgtcgggctccagacacttgaagatgactgagtagatactgacttcagggacctctccatggcttcgaccagctgctacacaagatgtgcccaggccagagagtaagtcatcagcaaaactcaggaattctcctgtgtacaggtcagtgtctgtgtattcatccactttcttatgctgcagaatatagtcggagaccttggtcccaatagctggctgaacatccacccactccaaggagaccacagtactggagggctccactgttggggacagccgcagcaccggctgcagaagggggctgcagttggggagcccattggcatcaaaggcgctgaggtcacacctgcaccagtcatcgatcacatcccctttccctgagcaccagtaggaactcatcagtgcactcttgaaggcctcctttgtgccattgtcttggatgagggtataaagtggcaccacacggttgatttccagcagcactggtgtggggctcagctgctccttgcctggccggcggcaaaggtgacaggtagatggacagcgccccttctcctcacagcgaatctccacacctgaaatgagctggtcatctgacagcatctgggctgtcagcaaacctgagaggtaggtgatgaagggcatggacttgagctccttcttgctgcccagctctgtggtctctttctgatactggagccacagctgctgctggaccttcttgctgggaaagtggatgatgcaggtgagctctgagccatagagggcctctgcgatgtagtgggagccatagtgctggatgaaggacagcagctcctcccgactgctctccttggtcaggatcttgagaacattagtgaagcctgctgcgagggtgatggtgctgagcttcacacggtagaggttgctccggacccgccactgctgcaccatggggtaacccatggcctcatcatacctgatatctccagtgagcagttggaggtctggaaggggctcggagaggaccccccggcactgctcctccaccggcagcgggatcaccaacagcccatcggccagctggggaaagtccttgatgaagttgttctccctaaaggtcatctggaagacttggccttggttcacatgctgggtccggttgttgtaaccatgtagcatctctccaaagagggtatcattgaatttggagtcaggtttgaggcacttggggccctcgcagacatctgagagcattaagcaggattttccatcaggagccagtttgtactcctccacgcaaccgcagaacatgaagatggtgctcgaagtggcatcgtagggcaggggcagcgtctgctgcaggcacagctgctcacagccgccattaaagccatcagagcagtcaatgcctttggagtggtcgtagcagccagagccatccttcatgggtttcagctcctcagggcacacacatcccgaggaatccacctgccggtcagacacacacttgaagttgcgagtgcagcccccattgttccgagagcagtcacgaactggcccgaaggaagacagcaggtcattgatggtttcaaagtatgtggacagcatcgcttcttccctgacatctgcagggtcttccgtgacgagcacatcggtcttgcagctggccagggggttgatggacagctccacaggcggaaccacaaagcttttgctgacaggaagccagaggccttggcccaagctgaaagtagacctgagaatcttttcaggggcttgctcccctgtcaccagatcatagcccctctcaagtgtcgtgtagggccaaggtccttcactctgtccccagtcactgcgcacacacaggtgtctgtgaacagggtcaggggcatagccttcatgacagctgcactctccggtttctgggtcgcagagctgctcacaggcatctgtcgtcctttgtccacagaggtccctcacccatggggaggtggcattgatctggtaatacagggaaagcttggccgggtttaaccagtcggagatgtccaggtagctcccttcactcaccacgaagctgcttccatctgctatgaagtgctcgggcacatgcagagtcaccttcacagtgagtggacaagacatctggctgccacacaccatggccaggatgcaggaactcacagcaatcagtgtcagggctgtcttgttcactgggcttttcagcaaacctttgctgcggcggcgactgcggtactgctccgtgtagaatgtcagctgagtttcatcgtctgcctctgagcccgacgtccccttggctctcccaaagctgattcctcctttcttctcaaagtccaccttctcttcccctggatgtcccagactgtccagagtgtgggtcacctggctgccaaactcgtcctcgcgggagacatggttggcccgcctaggtggctcctcatcctcctcacagtcatagtcatccaggatgggagtctcccggatgggcacgccaatgacggaattgtgggtttgcagccgggatgaacggaagctctcccgcgcctggggacccagcagcacagatgggatgtagtggatctcatgagtggcttctgtgcttgcgctcttctgggggatgcggcgacgcttctgccaacgtcgctgggcgtacagcgccacggtgaacaccagcagcagcagcagcagcgcgatgaggccacccatcacagaaatgtggaggatgtgcatctgctcctcaacaatctccgagggctcctggagagtgggggcggtggcttgggccagctgcccggagctgctcatggagacgtggaagtacaaggtgccattctccagccactgctgtctccagtgcaccagcgagatgtccgctgctgtgccagacatctccagggtgaagaagggcagctcggtgttgtccaggtcgtcctgcaccgcgatgcgccccggcagctcgttacgcacaaagagcaggaggcgcgactcggcggcggtgccggcagagccaggagagcccggggacgcggcggcggcggcggctccggccccggtcccagccccggccccggcgcgggcgccgctccagccgatgtcgctctcccgcagggcgggcagtgtggacaccgtgacggtcttcagccggcacgggctgtcgggctcccgcgaggcagcggcggtggcgccggccagcagcggcggcggcggcagcaggagcaggaacagcagcagcagcggcagcagtggcggcggccccgggtggaagcagagcctcggccgcccccggagccccgagccggggccggggctgagccgggcgccggcggcggccatggcgggaggggctgcggtgctgcgggcggcggcggcggtggcggcggtggcgaaggaggaagaggaggcagctgcggagacggcggacgccgaagcgaaccaggacgcccgagctaagg

SEQ ID NO: 15733 - RNA, 5124 nt, Homo sapiens
  source 1..5124: mol_type = other RNA
gctgggattacaggcatgagccactgtgcctggcaagcaaatcccatctttttcacctctctgtctggcttatttctactcatcctttgggtttaggtatcactttttcaaggaagcatttcaggagccctccagtgtgtctcatgctctaacagtgagtgcaaagaacctccattcttcctctagcacagcttgaaatgaccagactccttctctataatttccactgggcaataagttccctgagggaaggaagcttctctgtctttagttgcatatgctctgtgactggcacagggtagatactcaataagtgaataaacagaggtctctcaagcacattcccttggtaagaaataccacccaagcagaaagagagacaataggaatttttaatgcatggacaggcctgcagggactctgggcagacccacaggtagcaggaagaggcagggtcccacaaactcaataatgtccagcaaaaaagagagagaagtccttaaagacccatgcttcctcactgcaaccatcctcagagcttccttcctggtgctgaagaggtcaaaactgtctcctctaggggtcaggtcaaaactgtccctccataggtctcctccaggggtccatggcaggaagaaagcagagtgtggcaggaagaaggaagaagagcaaaggccgcttggtctccacctgaaaacttctgcctcgggattgacagccatccataagaaaaggtttaaaaaggagagacttttgatagagtcaaataatatctttgaaaaaataaaagatagagaaaaatgaataattccattggttacaaaggtctctgtccactatccacaggagaaaccgtttgctttggccttgctggcaagcttcatctgctaggcccatcctcagctgtcccccagcccacccaggccccaggatccaggagaatactgctccccctcccatggagagtctctgtgctcacggagggcaataccctccctcaccggcccttggactccccgtacgtgtttcgggccattgacaccatcttctcctcacacgtgattttggtgtccttgaggatgctataccacaccatgcctgcaggccggacctcctcgctgcggcagaaaagatagggcactgtttccacgcggctctggatgtaggcactccgcaggaggctggagcagtggctactcaccctctccagtcgccgtagaatcaggtgggccttcctgggccccagctcatcctcacttctccagacgaagtcgccaaacttttcatagtgagagttgtagtggtgctggactcggaacagcatcgaggctgagacctccatcagtgtgttgtaggccatctgctgctcctttccacttgtgtacccattgtacagattgtagatcttgtcagctatttcttctgccttgttgtcatctaccagtggacaggccgtcctcagggtcaccgtgcttagctctgagtgcctccctcgtgtatccacagcatacagagtgaacttgtagagaccgtcgggctccagacacttgaagatgactgagtagatactgacttcagggacctctccatggcttcgaccagctgctacacaagatgtgcccaggccagagagtaagtcatcagcaaaactcaggaattctcctgtgtacaggtcagtgtctgtgtattcatccactttcttatgctgcagaatatagtcggagaccttggtcccaatagctggctgaacatccacccactccaaggagaccacagtactggagggctccactgttggggacagccgcagcaccggctgcagaagggggctgcagttggggagcccattggcatcaaaggcgctgaggtcacacctgcaccagtcatcgatcacatcccctttccctgagcaccagtaggaactcatcagtgcactcttgaaggcctcctttgtgccattgtcttggatgagggtataaagtggcaccacacggttgatttccagcagcactggtgtggggctcagctgctccttgcctggccggcggcaaaggtgacaggtagatggacagcgccccttctcctcacagcgaatctccacacctgaaatgagctggtcatctgacagcatctgggctgtcagcaaacctgagaggtaggtgatgaagggcatggacttgagctccttcttgctgcccagctctgtggtctctttctgatactggagccacagctgctgctggaccttcttgctgggaaagtggatgatgcaggtgagctctgagccatagagggcctctgcgatgtagtgggagccatagtgctggatgaaggacagcagctcctcccgactgctctccttggtcaggatcttgagaacattagtgaagcctgctgcgagggtgatggtgctgagcttcacacggtagaggttgctccggacccgccactgctgcaccatggggtaacccatggcctcatcatacctgatatctccagtgagcagttggaggtctggaaggggctcggagaggaccccccggcactgctcctccaccggcagcgggatcaccaacagcccatcggccagctggggaaagtccttgatgaagttgttctccctaaaggtcatctggaagacttggccttggttcacatgctgggtccggttgttgtaaccatgtagcatctctccaaagagggtatcattgaatttggagtcaggtttgaggcacttggggccctcgcagacatctgagagcattaagcaggattttccatcaggagccagtttgtactcctccacgcaaccgcagaacatgaagatggtgctcgaagtggcatcgtagggcaggggcagcgtctgctgcaggcacagctgctcacagccgccattaaagccatcagagcagtcaatgcctttggagtggtcgtagcagccagagccatccttcatgggtttcagctcctcagggcacacacatcccgaggaatccacctgccggtcagacacacacttgaagttgcgagtgcagcccccattgttccgagagcagtcacgaactggcccgaaggaagacagcaggtcattgatggtttcaaagtatgtggacagcatcgcttcttccctgacatctgcagggtcttccgtgacgagcacatcggtcttgcagctggccagggggttgatggacagctccacaggcggaaccacaaagcttttgctgacaggaagccagaggccttggcccaagctgagaatcttttcaggggcttgctcccctgtcaccagatcatagcccctctcaagtgtcgtgtagggccaaggtccttcactctgtccccagtcactgcgcacacacaggtgtctgtgaacagggtcaggggcatagccttcatgacagctgcactctccggtttctgggtcgcagagctgctcacaggcatctgtcgtcctttgtccacagaggtccctcacccatggggaggtggcattgatctggtaatacagggaaagcttggccgggtttaaccagtcggagatgtccaggtagctcccttcactcaccacgaagctgcttccatctgctatgaagtgctcgggcacatgcagagtcaccttcacagtgagtggacaagacatctggctgccacacaccatggccaggatgcaggaactcacagcaatcagtgtcagggctgtcttgttcactgggcttttcagcaaacctttgctgcggcggcgactgcggtactgctccgtgtagaatgtcagctgagtttcatcgtctgcctctgagcccgacgtccccttggctctcccaaagctgattcctcctcgagacttgctcctccgcttcctcttccctgccgatgtgctgcgcaggggtggttgcagctgaccgatctcgatgggcgtgttagcgcggaaactctccttgaacttctgcatcagggactccactgtctcctgagtcgcctcagctgctgctttcttctcaaagtccaccttctcttcccctggatgtcccagactgtccagagtgtgggtcacctggctgccaaactcgtcctcgcgggagacatggttggcccgcctaggtggctcctcatcctcctcacagtcatagtcatccaggatgggagtctcccggatgggcacgccaatgacggaattgtgggtttgcagccgggatgaacggaagctctcccgcgcctggggacccagcagcacagatgggatgtagtggatctcatgagtggcttctgtgcttgcgctcttctgggggatgcggcgacgcttctgccaacgtcgctgggcgtacagcgccacggtgaacaccagcagcagcagcagcagcgcgatgaggccacccatcacagaaatgtggaggatgtgcatctgctcctcaacaatctccgagggctcctggagagtgggggcggtggcttgggccagctgcccggagctgctcatggagacgtggaagtacaaggtgccattctccagccactgctgtctccagtgcaccagcgagatgtccgctgctgtgccagacatctccagggtgaagaagggcagctcggtgttgtccaggtcgtcctgcaccgcgatgcgccccggcagctcgttacgcacaaagagcaggaggcgcgactcggcggcggtgccggcagagccaggagagcccggggacgcggcggcggcggcggctccggccccggtcccagccccggccccggcgcgggcgccgctccagccgatgtcgctctcccgcagggcgggcagtgtggacaccgtgacggtcttcagccggcacgggctgtcgggctcccgcgaggcagcggcggtggcgccggccagcagcggcggcggcggcagcaggagcaggaacagcagcagcagcggcagcagtggcggcggccccgggtggaagcagagcctcggccgcccccggagccccgagccggggccggggctgagccgggcgccggcggcggccatggcgggaggggctgcggtgctgcgggcggcggcggcggtggcggcggtggcgaaggaggaagaggaggcagctgcggagacggcggacgccgaagcgaaccaggacgcccgagctaagg

SEQ ID NO: 15734 - RNA, 2755 nt, Homo sapiens
  source 1..2755: mol_type = other RNA
gctgggattacaggcatgagccactgtgcctggcagaaaagctgtcagagagactcctgggtcccaccgtagggggaaaagggcctttactgctcaagggaactggcgctgcccatggcccagtgtacaagctccctactcacagggcctatctatgggaagcccctttctgggcccacctcccatgggtgcctgtgtcaccaggcttccttggctttgaggacccctgcccagtgggggaggaccctggggactctcaaggccaaactcactttagggatgaatcatgacgtgcagtttggaggcctgcatggctcatcacccggtgggaagcagtgcttgggttgcttgccctggatggcaccctacagagacccaggggtgggacacaggactgcaggggaaggccgccttcctgagggcagggtcttaggggccgcacatttactctaagggcactgttacggttcataccactcctgggctccttgctgcacagcacccttggagaccgtctctttcctctggatctcctcaggggccgtgaatcttcctcttccagcagaaaatggtcgaaaggtatatggagccacagatggtggggaaggtgggtgaagtgggggtcacaaacgaggtgaagctacaacaaaaggggactgacttacaggggatagaaaagagctaactttgattctgaagacagatcccagaggggaatctgaattctgagtaatgatgttttcagaaaaatgtctggtctctcaaggtgactattttgaaagcaaagatatataactgggtgaatgggaaggtctgcaaccaagatccagcaagtggcaggacagattttggctcaatatagggaagaactgtctaacagtcagcactgtccaaccacagcaggagctgccttggggatggcgcgcttcctatcagccaaggtatgcaagcaggccaaggtgatcacttgcaggtacccagggagaggcgctcatcttcagatgtgctggggtgttctaggggtgggggaggactaagcaatcatcgaattatttccaaccctgagaatccgtaatagatttgtttaaaatgacctgtttcaatgatacctcaaatttttgggaaaacaatgacaaaagtcaggtaacaggctggatttggaagtgatttcattacactggctacagatacttgcacatttttgcaaagatagcagaccctttctaaagccaggaatcccttgattcagccctatcaagagggacattcctaccttctgaactctgcctggacactcattcctctagaccctgccacacctcatctctgacccccaagaggggacactaacagagctctgagaatgcacagcattccaagccagccaaacatggtcacccctgggcaaacatccacgatcatggatgcaccctggggagggaggagcaggtgtgacaggaaccgctggggactttatgtcctggttaactggaggtagcctcttgttctcatcccatcctctccaccagggccttcttacagatggataaatgcggcactggctagcggtacagagagatggagcccaggagaaaactgctgctcttttgtcctggctggaaaatcctcctatggcctcctttagtacacatcagctgactcttcacttgtcataataaaccgcctgtctgcagctcaaaatggcaagaaaaaaggtggttctgttcagaggacactggattccaaaaggtggacttcatcatggggggaatcaagtcctgctacacaattaatacagattagtatagtcccctgcctcgcaccactggcgagatgccctccaagacctggctgacatgagcttcctgggactccccatctccagtgttgttggggtccttttacctgtaccgtattaatcgaataatcttattgttcataaaatccagagcatgtgggtgagaagaatcgatgcagaagccatcgctcagagcgattttcagtacctcttccacgaagacctggaagctgttgatctgcttgttggcgggcaccacccagagcctcttgaggttctgcttggtgtactcctcctctggcaggccctccacattggccacccagtccagagtcaggtggttggggtcctgcaagtggctggtgatggaggagagattgccattggagcagtagaagagcttagagccaaggagcttgaggaagaggcaggaggtgctgaagatgttggcgttgaagacctccatgctggaagaggagaggctgtagatctggggtgcctcgcgcacagtgaagtggaccgtctgcacacgctggttcagtgtgatgttgagcatggcattcttctcggccttggagagctccacttccttctcctgcagggcctcaatcaggggctgcacctggtagaagtcggcctccctgcggagcagccccatctcctggaagtcctcaggcaggtcaaggtgggaggtccgcaggaagttgaggatatagcggaacactttgccgtcacggtcaatgaagcagttgccctggctgtccctcttggtgggcatcttcccgctgaacatggcgcctagcatggagtcagggaagctggtcagggtcgccagtgaggttgtatagagcttccccccgacgttcagcgtgatggggtcggacatggcaggagactgggttgctggaagtagtccctcgccggtagtccccgagccccgcgaccccggccgtgccg

SEQ ID NO: 15735 - RNA, 5940 nt, Homo sapiens
  source 1..5940: mol_type = other RNA
gctgggattacaggcatgagccactgtgcctggcagaaaagctgtcagagagactcctgggtcccaccgtagggggaaaagggcctttactgctcaagggaactggcgctgcccatggcccagtgtacaagctccctactcacagggcctatctatgggaagcccctttctgggcccacctcccatgggtgcctgtgtcaccaggcttccttggctttgaggacccctgcccagtgggggaggaccctggggactctcaaggccaaactcactttagggatgaatcatgacgtgcagtttggaggcctgcatggctcatcacccggtgggaagcagtgcttgggttgcttgccctggatggcaccctacagagacccaggggtgggacacaggactgcaggggaaggccgccttcctgagggcagggtcttaggggccgcacatttactctaagggcactgttacggttcataccactcctgggctccttgctgcacagcacccttggagaccgtctctttcctctggatctcctcaggggccgtgaatcttcctcttccagcagaaaatggtcgaaaggtatatggagccacagatggtggggaaggtgggtgaagtgggggtcacaaacgaggtgaagctacaacaaaaggggactgacttacaggggatagaaaagagctaactttgattctgaagacagatcccagaggggaatctgaattctgagtaatgatgttttcagaaaaatgtctggtctctcaaggtgactattttgaaagcaaagatatataactgggtgaatgggaaggtctgcaaccaagatccagcaagtggcaggacagattttggctcaatatagggaagaactgtctaacagtcagcactgtccaaccacagcaggagctgccttggggatggcgcgcttcctatcagccaaggtatgcaagcaggccaaggtgatcacttgcaggtacccagggagaggcgctcatcttcagatgtgctggggtgttctaggggtgggggaggactaagcaatcatcgaattatttccaaccctgagaatccgtaatagatttgtttaaaatgacctgtttcaatgatacctcaaatttttgggaaaacaatgacaaaagtcaggtaacaggctggatttggaagtgatttcattacactggctacagatacttgcacatttttgcaaagatagcagaccctttctaaagccaggaatcccttgattcagccctatcaagagggacattcctaccttctgaactctgcctggacactcattcctctagaccctgccacacctcatctctgacccccaagaggggacactaacagagctctgagaatgcacagcattccaagccagccaaacatggtcacccctgggcaaacatccacgatcatggatgcaccctggggagggaggagcaggtgtgacaggaaccgctggggactttatgtcctggttaactggaggtagcctcttgttctcatcccatcctctccaccagggccttcttacagatggataaatgcggcactggctagcggtacagagagatggagcccaggagaaaactgctgctcttttgtcctggctggaaaatcctcctatggcctcctttagtacacatcagctgactcttcacttgtcataataaaccgcctgtctgcagctcaaaatggcaagaaaaaaggtggttctgttcagaggacactggattccaaaaggtggacttcatcatggggggaatcaagtcctgctacacaattaatacagattagtatagtcccctgcctcgcaccactggcgagatgccctccaagacctggctgacatgagcttcctgggactccccatctccagtgttgttggggtccttttacctgtaccgtattaatcgaataatcttattgttcataaaatccagagcatgtgggtgagaagaatcgatgcagaagccatcgctcagagcgattttcagtacctcttccacgaagacctggaagctgttgatctgcttgttggcgggcaccacccagagcctcttgaggttctgcttggtgtactcctcctctggcaggccctccacattggccacccagtccagagtcaggtggttggggtcctgcaagtggctggtgatggaggagagattgccattggagcagtagaagagcttagagccaaggagcttgaggaagaggcaggaggtgctgaagatgttggcgttgaagacctccatgctggaagaggagaggctgtagatctggggtgcctcgcgcacagtgaagtggaccgtctgcacacgctggttcagtgtgatgttgagcatggcattcttctcggccttggagagctccacttccttctcctgcagggcctcaatcaggggctgcacctggtagaagtcggcctccctgcggagcagccccatctcctggaagtcctcaggcaggtcaaggtgggaggtccgcaggaagttgaggatatagcggaacactttgccgtcacggtcaatgaagcagttgccctggctgtccctcttggtgggcatcttcccgctgaacatggcgcctagcatggagtcagggaagctggtcagggtcgccagtgaggttgtatagagcttccccccgacgttcagcgtgatggggtcggacatggcaggagactgggttgctggaagtagtccgtccagatggagaaacagaggtctgaggagacacctccccaaagtcacccagcaggggtggcgagaacttctcaacatttctgcctcctgaagaggctgactgcactgaggcctcctttctccagaggatgggggccatgccagtgtgagagatattcagctgccatgctcgactctgtggcaggggcaggggtatgtcccctcatgattcctccccagtctaatggggcactttgatattgcagaaaggcattccccatctggagtgtctgaggagaaatgagtccatgtgaaatacgaaatcgtcagtagaagcctggagcagatgggctgcgagacggtggggaggtcccacagaggtgtgggcgagctgccgctgggggcatggctgctggtgtggagatggctgtgaggcagcaactggggagggtgctgtgactcagggctgaatctggccaattctctctccagagggcccaggcaggaggtggacccaggagtgggtcccctttactcagtccagaatcttcttccctgttgccctctttgtaggactctagtctactccaactgttttcttctggatagaaatgtgcatgttctagtttcagtctctctttcttcttgaaaacaaacactccctcccaacattgggtttcaggcctaggatctataaagtggcttaccttcacggcaggaaaagaagcgggtgtcagagaggacttggacagttccatgggtcacagacccttatctcttccatgcattactgctgaagtgctcagagcattacaggcgggggaggtcaggagccacagggcattccctgggacccctgggtaggtgcccaaactcttatttctctgcttgcaaaagcagcagagcacctgctttcctgcgcccccgatgacgtcatggctcccggtcatttgtctggggagagcagcacagttgcacaggcagtcagggcagaggctggctagcaggcaggtctcctgctccgagtctagggtgctctctgtggtgatctccccttacctatccagtcacagagctcagtcctctaagcccttcttttctttttttttttttgagatggagtctcgctctgtcgccaggctagagtgcagtgacgcaatctcagctcactgcaacctctgcctcccagattcaagcgacactcctgcctcagcctcccgggtagctgcaattacaggtgcacgccaccaggcccggctaatttatttttgtatttttagtagagatgggatttcaccatgttggccaggatggtctcgatctcttgactttgtgatctgcccgcctcggcctcccaaagtgctgggattacaggcgtgagccaccgtgcctggtctaagcccctattttctagccacagggccacagtgtccatcatcacaaatccacggccctgctacaaaaggcaaaatgacatgacacgaggggagtttcatgagtcggcggaggtttgcagtcaggtagtaatgaactaacaccactgagcctcagtcccctatgtgttcccagatgcctcctggccacctccacttggatattctgcaagtgaggcaggagaacaaggtttggagacaaggaacttaaggccaatttgtgctaacttcataaaagagaaaacaccaaggtctggggcaaaaaatctgaggccaattctgttgacttcccaaagctggatcagaaggaaaatcctgggtctgggggcagggaccctaagaccaattaacaccaaattcctaaagctgaaccaagaggaaaaacgccatcgccccagctgggtgacaaaggatcaaacgctcctctttgcaaccctcccactccaccatgtctcaggtggaaagggaggggggccttggattgggaccatccctttatctgcatagggtgcccattcacctcagcctttaattagccacagactaaatccttcgtccagataaggagtagctgataagaacctcaaatggggtacctaaagcccagagaactttgtaactgggcctttgagttccttgctccggcccactcccaccctgaggagtgctttctcactttaattcctgctttcactgcttcattcctgcatttcattcccctgctactctttttatttttactttttttttttttagtagagacgggtttcaccacgttggccaggccggtcttggactgacctcaagtgatctgcccatccaggcctcccaaagtgtggggattaccacgtctgcccctctgctactttgttcaaaacgccaaggacctggaaaattcctagtcaagaccctccaccagtaacacaggtaccagaagcctcacctgtgccttcctctgcccctaactctgctgtgaactcttctgagccacccaactgcctgagggaagcagccccgactcttcagccctacagtttgtcttgactatctccttgaacccatccctatagctactcccagagctcaggcctcatccctgccccctgcacccctacatcctcactcggctccctgccttctgtccaccttcctttctggtctgcagactgaccttcctgaagtaccgtccctgcccaaccaccttcctctttccctctcatgtctaaccctgccctccacgcacgccagacgccactgagtcagtctccttcatgctgacacctgccctgcctttgctgtccctagaccacccctgtctaccttctctaccctctctgctgtctacctttcaggcccagcctatgagtcatcacctctgtactactgtccccagatctccactaggttaacagctctcctctcagggcttcctggtgccttgcacaaccccctctggcagcacccagcattccacctgcagcgatctcctttgcacatggccctcttccctggctatctcaaaatgcagatcagtggacatccatatggggaaaaaaagaaccttggtccatctcttatgctgtttatgaaaaataaactcagaacatatcatagacctaaatataaaatctaaaactacacaacttctaggagaaaatctttgcaactgtggattaggcaaagatttcttggataggacctaaaagggacaaaccattaaaaacatcaataaactagacttcatccacgtaaaaaacttctgctcttcaaaagacactgttaagaaaatgaaagaataagacacagatggagaa

SEQ ID NO: 15736 - RNA, 2767 nt, Homo sapiens
  source 1..2767: mol_type = other RNA
gctgggattacaggcatgagccactgtgcctggcagaaaagctgtcagagagactcctgggtcccaccgtagggggaaaagggcctttactgctcaagggaactggcgctgcccatggcccagtgtacaagctccctactcacagggcctatctatgggaagcccctttctgggcccacctcccatgggtgcctgtgtcaccaggcttccttggctttgaggacccctgcccagtgggggaggaccctggggactctcaaggccaaactcactttagggatgaatcatgacgtgcagtttggaggcctgcatggctcatcacccggtgggaagcagtgcttgggttgcttgccctggatggcaccctacagagacccaggggtgggacacaggactgcaggggaaggccgccttcctgagggcagggtcttaggggccgcacatttactctaagggcactgttacggttcataccactcctgggctccttgctgcacagcacccttggagaccgtctctttcctctggatctcctcaggggccgtgaatcttcctcttccagcagaaaatggtcgaaaggtatatggagccacagatggtggggaaggtgggtgaagtgggggtcacaaacgaggtgaagctacaacaaaaggggactgacttacaggggatagaaaagagctaactttgattctgaagacagatcccagaggggaatctgaattctgagtaatgatgttttcagaaaaatgtctggtctctcaaggtgactattttgaaagcaaagatatataactgggtgaatgggaaggtctgcaaccaagatccagcaagtggcaggacagattttggctcaatatagggaagaactgtctaacagtcagcactgtccaaccacagcaggagctgccttggggatggcgcgcttcctatcagccaaggtatgcaagcaggccaaggtgatcacttgcaggtacccagggagaggcgctcatcttcagatgtgctggggtgttctaggggtgggggaggactaagcaatcatcgaattatttccaaccctgagaatccgtaatagatttgtttaaaatgacctgtttcaatgatacctcaaatttttgggaaaacaatgacaaaagtcaggtaacaggctggatttggaagtgatttcattacactggctacagatacttgcacatttttgcaaagatagcagaccctttctaaagccaggaatcccttgattcagccctatcaagagggacattcctaccttctgaactctgcctggacactcattcctctagaccctgccacacctcatctctgacccccaagaggggacactaacagagctctgagaatgcacagcattccaagccagccaaacatggtcacccctgggcaaacatccacgatcatggatgcaccctggggagggaggagcaggtgtgacaggaaccgctggggactttatgtcctggttaactggaggtagcctcttgttctcatcccatcctctccaccagggccttcttacagatggataaatgcggcactggctagcggtacagagagatggagcccaggagaaaactgctgctcttttgtcctggctggaaaatcctcctatggcctcctttagtacacatcagctgactcttcacttgtcataataaaccgcctgtctgcagctcaaaatggcaagaaaaaaggtggttctgttcagaggacactggattccaaaaggtggacttcatcatggggggaatcaagtcctgctacacaattaatacagattagtatagtcccctgcctcgcaccactggcgagatgccctccaagacctggctgacatgagcttcctgggactccccatctccagtgttgttggggtccttttacctgtaccgtattaatcgaataatcttattgttcataaaatccagagcatgtgggtgagaagaatcgatgcagaagccatcgctcagagcgattttcagtacctcttccacgaagacctggaagctgttgatctgcttgttggcgggcaccacccagagcctcttgaggttctgcttggtgtactcctcctctggcaggccctccacattggccacccagtccagagtcaggtggttggggtcctgcaagtggctggtgatggaggagagattgccattggagcagtagaagagcttagagccaaggagcttgaggaagaggcaggaggtgctgaagatgttggcgttgaagacctccatgctggaagaggagaggctgtagatctggggtgcctcgcgcacagtgaagtggaccgtctgcacacgctggttcagtgtgatgttgagcatggcattcttctcggccttggagagctccacttccttctcctgcagggcctcaatcaggggctgcacctggtagaagtcggcctccctgcggagcagccccatctcctggaagtcctcaggcaggtcaaggtgggaggtccgcaggaagttgaggatatagcggaacactttgccgtcacggtcaatgaagcagttgccctggctgtccctcttggtgggcatcttcccgctgaacatggcgcctagcatggagtcagggaagctggtcagggtcgccagtgaggttgtatagagcttccccccgacgttcagcgtgatggggtcggacatggcaggagactgggttgctggaagtagtcctcctgccctcgctctgcagcctctccctccgcgagcggccagcgcagctttgc

SEQ ID NO: 15737 - RNA, 3007 nt, Homo sapiens
  source 1..3007: mol_type = other RNA
gctgggattacaggcatgagccactgtgcctggcagaaaagctgtcagagagactcctgggtcccaccgtagggggaaaagggcctttactgctcaagggaactggcgctgcccatggcccagtgtacaagctccctactcacagggcctatctatgggaagcccctttctgggcccacctcccatgggtgcctgtgtcaccaggcttccttggctttgaggacccctgcccagtgggggaggaccctggggactctcaaggccaaactcactttagggatgaatcatgacgtgcagtttggaggcctgcatggctcatcacccggtgggaagcagtgcttgggttgcttgccctggatggcaccctacagagacccaggggtgggacacaggactgcaggggaaggccgccttcctgagggcagggtcttaggggccgcacatttactctaagggcactgttacggttcataccactcctgggctccttgctgcacagcacccttggagaccgtctctttcctctggatctcctcaggggccgtgaatcttcctcttccagcagaaaatggtcgaaaggtatatggagccacagatggtggggaaggtgggtgaagtgggggtcacaaacgaggtgaagctacaacaaaaggggactgacttacaggggatagaaaagagctaactttgattctgaagacagatcccagaggggaatctgaattctgagtaatgatgttttcagaaaaatgtctggtctctcaaggtgactattttgaaagcaaagatatataactgggtgaatgggaaggtctgcaaccaagatccagcaagtggcaggacagattttggctcaatatagggaagaactgtctaacagtcagcactgtccaaccacagcaggagctgccttggggatggcgcgcttcctatcagccaaggtatgcaagcaggccaaggtgatcacttgcaggtacccagggagaggcgctcatcttcagatgtgctggggtgttctaggggtgggggaggactaagcaatcatcgaattatttccaaccctgagaatccgtaatagatttgtttaaaatgacctgtttcaatgatacctcaaatttttgggaaaacaatgacaaaagtcaggtaacaggctggatttggaagtgatttcattacactggctacagatacttgcacatttttgcaaagatagcagaccctttctaaagccaggaatcccttgattcagccctatcaagagggacattcctaccttctgaactctgcctggacactcattcctctagaccctgccacacctcatctctgacccccaagaggggacactaacagagctctgagaatgcacagcattccaagccagccaaacatggtcacccctgggcaaacatccacgatcatggatgcaccctggggagggaggagcaggtgtgacaggaaccgctggggactttatgtcctggttaactggaggtagcctcttgttctcatcccatcctctccaccagggccttcttacagatggataaatgcggcactggctagcggtacagagagatggagcccaggagaaaactgctgctcttttgtcctggctggaaaatcctcctatggcctcctttagtacacatcagctgactcttcacttgtcataataaaccgcctgtctgcagctcaaaatggcaagaaaaaaggtggttctgttcagaggacactggattccaaaaggtggacttcatcatggggggaatcaagtcctgctacacaattaatacagattagtatagtcccctgcctcgcaccactggcgagatgccctccaagacctggctgacatgagcttcctgggactccccatctccagtgttgttggggtccttttacctgtaccgtattaatcgaataatcttattgttcataaaatccagagcatgtgggtgagaagaatcgatgcagaagccatcgctcagagcgattttcagtacctcttccacgaagacctggaagctgttgatctgcttgttggcgggcaccacccagagcctcttgaggttctgcttggtgtactcctcctctggcaggccctccacattggccacccagtccagagtcaggtggttggggtcctgcaagtggctggtgatggaggagagattgccattggagcagtagaagagcttagagccaaggagcttgaggaagaggcaggaggtgctgaagatgttggcgttgaagacctccatgctggaagaggagaggctgtagatctggggtgcctcgcgcacagtgaagtggaccgtctgcacacgctggttcagtgtgatgttgagcatggcattcttctcggccttggagagctccacttccttctcctgcagggcctcaatcaggggctgcacctggtagaagtcggcctccctgcggagcagccccatctcctggaagtcctcaggcaggtcaaggtgggaggtccgcaggaagttgaggatatagcggaacactttgccgtcacggtcaatgaagcagttgccctggctgtccctcttggtgggcatcttcccgctgaacatggcgcctagcatggagtcagggaagctggtcagggtcgccagtgaggttgtatagagcttccccccgacgttcagcgtgatggggtcggacatggcaggagactgggttgctggaagtagtccttcacggcaggaaaagaagcgggtgtcagagaggacttggacagttccatgggtcacagacccttatctcttccatgcattactgctgaagtgctcagagcattacaggcgggggaggtcaggagccacagggcattccctgggacccctgggtaggtgcccaaactcttatttctctgcttgcaaaagcagcagagcacctgctttcctgcgcccccgatgacgtcatggctcccggtcatttgtctcctgccctcgctctgcagcctctccctccgcgagcggccagcgca

SEQ ID NO: 15738 - RNA, 2895 nt, Homo sapiens
  source 1..2895: mol_type = other RNA
gctgggattacaggcatgagccactgtgcctggcagaaaagctgtcagagagactcctgggtcccaccgtagggggaaaagggcctttactgctcaagggaactggcgctgcccatggcccagtgtacaagctccctactcacagggcctatctatgggaagcccctttctgggcccacctcccatgggtgcctgtgtcaccaggcttccttggctttgaggacccctgcccagtgggggaggaccctggggactctcaaggccaaactcactttagggatgaatcatgacgtgcagtttggaggcctgcatggctcatcacccggtgggaagcagtgcttgggttgcttgccctggatggcaccctacagagacccaggggtgggacacaggactgcaggggaaggccgccttcctgagggcagggtcttaggggccgcacatttactctaagggcactgttacggttcataccactcctgggctccttgctgcacagcacccttggagaccgtctctttcctctggatctcctcaggggccgtgaatcttcctcttccagcagaaaatggtcgaaaggtatatggagccacagatggtggggaaggtgggtgaagtgggggtcacaaacgaggtgaagctacaacaaaaggggactgacttacaggggatagaaaagagctaactttgattctgaagacagatcccagaggggaatctgaattctgagtaatgatgttttcagaaaaatgtctggtctctcaaggtgactattttgaaagcaaagatatataactgggtgaatgggaaggtctgcaaccaagatccagcaagtggcaggacagattttggctcaatatagggaagaactgtctaacagtcagcactgtccaaccacagcaggagctgccttggggatggcgcgcttcctatcagccaaggtatgcaagcaggccaaggtgatcacttgcaggtacccagggagaggcgctcatcttcagatgtgctggggtgttctaggggtgggggaggactaagcaatcatcgaattatttccaaccctgagaatccgtaatagatttgtttaaaatgacctgtttcaatgatacctcaaatttttgggaaaacaatgacaaaagtcaggtaacaggctggatttggaagtgatttcattacactggctacagatacttgcacatttttgcaaagatagcagaccctttctaaagccaggaatcccttgattcagccctatcaagagggacattcctaccttctgaactctgcctggacactcattcctctagaccctgccacacctcatctctgacccccaagaggggacactaacagagctctgagaatgcacagcattccaagccagccaaacatggtcacccctgggcaaacatccacgatcatggatgcaccctggggagggaggagcaggtgtgacaggaaccgctggggactttatgtcctggttaactggaggtagcctcttgttctcatcccatcctctccaccagggccttcttacagatggataaatgcggcactggctagcggtacagagagatggagcccaggagaaaactgctgctcttttgtcctggctggaaaatcctcctatggcctcctttagtacacatcagctgactcttcacttgtcataataaaccgcctgtctgcagctcaaaatggcaagaaaaaaggtggttctgttcagaggacactggattccaaaaggtggacttcatcatggggggaatcaagtcctgctacacaattaatacagattagtatagtcccctgcctcgcaccactggcgagatgccctccaagacctggctgacatgagcttcctgggactccccatctccagtgttgttggggtccttttacctgtaccgtattaatcgaataatcttattgttcataaaatccagagcatgtgggtgagaagaatcgatgcagaagccatcgctcagagcgattttcagtacctcttccacgaagacctggaagctgttgatctgcttgttggcgggcaccacccagagcctcttgaggttctgcttggtgtactcctcctctggcaggccctccacattggccacccagtccagagtcaggtggttggggtcctgcaagtggctggtgatggaggagagattgccattggagcagtagaagagcttagagccaaggagcttgaggaagaggcaggaggtgctgaagatgttggcgttgaagacctccatgctggaagaggagaggctgtagatctggggtgcctcgcgcacagtgaagtggaccgtctgcacacgctggttcagtgtgatgttgagcatggcattcttctcggccttggagagctccacttccttctcctgcagggcctcaatcaggggctgcacctggtagaagtcggcctccctgcggagcagccccatctcctggaagtcctcaggcaggtcaaggtgggaggtccgcaggaagttgaggatatagcggaacactttgccgtcacggtcaatgaagcagttgccctggctgtccctcttggtgggcatcttcccgctgaacatggcgcctagcatggagtcagggaagctggtcagggtcgccagtgaggttgtatagagcttccccccgacgttcagcgtgatggggtcggacatggcaggagactgggttgctggaagtagtctttacagaccaaccatactgggccctcttcgacttctgcaatttggcatctgccatcccctctgcctggaccttgaagacaaatcccatgcatcggccaggtctctcagctggaattcattccttctcctctgcatctcctgccctcgctctgcagcctctccctccgcgagcggccagcgc

SEQ ID NO: 15739 - RNA, 4234 nt, Homo sapiens
  source 1..4234: mol_type = other RNA
gctgggattacaggcatgagccactgtgcctggcagaaaagctgtcagagagactcctgggtcccaccgtagggggaaaagggcctttactgctcaagggaactggcgctgcccatggcccagtgtacaagctccctactcacagggcctatctatgggaagcccctttctgggcccacctcccatgggtgcctgtgtcaccaggcttccttggctttgaggacccctgcccagtgggggaggaccctggggactctcaaggccaaactcactttagggatgaatcatgacgtgcagtttggaggcctgcatggctcatcacccggtgggaagcagtgcttgggttgcttgccctggatggcaccctacagagacccaggggtgggacacaggactgcaggggaaggccgccttcctgagggcagggtcttaggggccgcacatttactctaagggcactgttacggttcataccactcctgggctccttgctgcacagcacccttggagaccgtctctttcctctggatctcctcaggggccgtgaatcttcctcttccagcagaaaatggtcgaaaggtatatggagccacagatggtggggaaggtgggtgaagtgggggtcacaaacgaggtgaagctacaacaaaaggggactgacttacaggggatagaaaagagctaactttgattctgaagacagatcccagaggggaatctgaattctgagtaatgatgttttcagaaaaatgtctggtctctcaaggtgactattttgaaagcaaagatatataactgggtgaatgggaaggtctgcaaccaagatccagcaagtggcaggacagattttggctcaatatagggaagaactgtctaacagtcagcactgtccaaccacagcaggagctgccttggggatggcgcgcttcctatcagccaaggtatgcaagcaggccaaggtgatcacttgcaggtacccagggagaggcgctcatcttcagatgtgctggggtgttctaggggtgggggaggactaagcaatcatcgaattatttccaaccctgagaatccgtaatagatttgtttaaaatgacctgtttcaatgatacctcaaatttttgggaaaacaatgacaaaagtcaggtaacaggctggatttggaagtgatttcattacactggctacagatacttgcacatttttgcaaagatagcagaccctttctaaagccaggaatcccttgattcagccctatcaagagggacattcctaccttctgaactctgcctggacactcattcctctagaccctgccacacctcatctctgacccccaagaggggacactaacagagctctgagaatgcacagcattccaagccagccaaacatggtcacccctgggcaaacatccacgatcatggatgcaccctggggagggaggagcaggtgtgacaggaaccgctggggactttatgtcctggttaactggaggtagcctcttgttctcatcccatcctctccaccagggccttcttacagatggataaatgcggcactggctagcggtacagagagatggagcccaggagaaaactgctgctcttttgtcctggctggaaaatcctcctatggcctcctttagtacacatcagctgactcttcacttgtcataataaaccgcctgtctgcagctcaaaatggcaagaaaaaaggtggttctgttcagaggacactggattccaaaaggtggacttcatcatggggggaatcaagtcctgctacacaattaatacagattagtatagtcccctgcctcgcaccactggcgagatgccctccaagacctggctgacatgagcttcctgggactccccatctccagtgttgttggggtccttttacctgtaccgtattaatcgaataatcttattgttcataaaatccagagcatgtgggtgagaagaatcgatgcagaagccatcgctcagagcgattttcagtacctcttccacgaagacctggaagctgttgatctgcttgttggcgggcaccacccagagcctcttgaggttctgcttggtgtactcctcctctggcaggccctccacattggccacccagtccagagtcaggtggttggggtcctgcaagtggctggtgatggaggagagattgccattggagcagtagaagagcttagagccaaggagcttgaggaagaggcaggaggtgctgaagatgttggcgttgaagacctccatgctggaagaggagaggctgtagatctggggtgcctcgcgcacagtgaagtggaccgtctgcacacgctggttcagtgtgatgttgagcatggcattcttctcggccttggagagctccacttccttctcctgcagggcctcaatcaggggctgcacctggtagaagtcggcctccctgcggagcagccccatctcctggaagtcctcaggcaggtcaaggtgggaggtccgcaggaagttgaggatatagcggaacactttgccgtcacggtcaatgaagcagttgccctggctgtccctcttggtgggcatcttcccgctgaacatggcgcctagcatggagtcagggaagctggtcagggtcgccagtgaggttgtatagagcttccccccgacgttcagcgtgatggggtcggacatggcaggagactgggttgctggaagtagtctttacagaccaaccatactgggccctcttcgacttctgcaatttggcatctgccatcccctctgcctggaccttgaagacaaatcccatgcatcggccaggtctctcagctggaattcattccttctcctctgcatctgcggagaattttagtctaaccccttaccacagccaactttacttaagtagatggatgcctggctcccttgctggggctgggggtgcccctttctatatccacagaagcacgtagaataggggaagaggaagaaatttctctcctgtttagtcagatccattttccccacctggattttcaaaactttttaattttgaaatgctctgttcaattttcaatctggaatctaaagggatgtgacaaggccgaggtgattacttgggagtaaatgcaaggagagtttccactgcgtaagggaatggacagcacgtggctgggtaaatttcaaaaaagacaatgctcagagtgagtactgtgttttccagtaagtgggagacttccccaccttaccccaccggagaaaggactctttgccttgaagcccctaggacgactaccctttcttcacctcctcttcctgaccaccccacatcaaagagctgcgtctataattctgtcttgcccagtccatatctctaagaaatccgaaggctgctctattaccatcacaacccatagggaggagagaaaaggtgcttcctagacacagggaccccagaatgagctgcgcaaaaggcaggaggagagaaaggtgggctggaagaaggagaccacggaatctggcacggcaaggtattctttcatctggcgtagacctccaacaaccactaccatcccccagccccttccagaactttccttcaccttctcggctcactctcacgcttcaccttgtgcttttcctccggcaccagcaccccatttcaaaccgctctcttcctatgtctcctccaaacagtaatttataaacaccgtgctttcaaatccatctcatttcatcctcacagtactataggagggctgccttacaggctgtcattcggaagggttggggggactggtcctgccagacaatttgcgaaggtcggggcatcaaaacttttctttcctgcctcccacgccaagctaaacctctgcctccccgagtgcagggagaaaagcaaggtctttgaagtaaggagtcctgagtggttttaggcaagtcccttcgcttttctgagcctcacattcctcacctgtcaaccgctatagtgacgcctctacttttcagggcgtgggaggtcaatgagatcactggtgtgccgcactgaactcggggatggactctttatttccagtcagtaaagggaggtgttctatgcatcacaggcttttgcccacgccgccacagcgcggccggcccagggctctccagagcggggcaagttccctgtcatctgtgtctccgcccttccttccccaatctcacccaggctggcctcatcggcttgttccgcacccact

SEQ ID NO: 15740 - RNA, 1537 nt, Homo sapiens
  source 1..1537: mol_type = other RNA
gctgggattacaggcatgagccactgtgcctggcagaggactgcatttttcgggagtttgtgtgttccatgtgtactccttgcactcacagcactgaaagtagtaagaagccacctggaagttttctgagatactcctgcaagaaagagcttggttgactcctcctgtttctgtttatctcgaaggctctgcagcaattttcccaaactgaacagcaagagggagacctcaaagaggcgactctcttcctagctgcatctccttcctaatcctctgggtgccttggaatagaagctcagaaggaagaaaacgacattttcaactttcaggaactagctctgtcgccctctgcacagctcgggagacagcactctcagccttttaggactccatccaaaaatccttcagccctccatgttccccaaaatgacagtgctcatgtgtggctggaacctgccccgatccggcagctcatttaaatagagctcatcacaacaacagtgttggtggtgaagtgagtagctgcaggaccctggggaccccctgtttatacgtaggaagaatgatgcaatctgggtatcaaaatagcaatccagaatggaataacaggctcacgcagcagcggtgcctgcacagccagagctcaagttgacacactctgtcagccccacactgctgcagcacgcagatgccaggcacacactctcaccgcatcattttaaaaaacagcaggagcccaagatatccctccatgcccccggcactgaaggagggtgtgggggggccttcaacagacattgaaatctgtctcctacatactcacctgctcctgccacttcacctgaagtccttatcctgtgacgtcacagtcagttgccatagtgaccaattgtccgtcacaagcagaggattaggacttcggatggagaagacacacatttacgatgcacaaaggtcctgggaggtctcccttggcagttaactctacccaccaggaagatccagtcacacacaagcagggagggaaaaagggaagaatgaacagggttgactggaggagacattaggatggggcaagactacaagtacagcataatttcaaaagcacagagcaaccagatgagggggagtggcagggatgtgcttggaaagaccggaaggagagtaagctcctgaagggacctgaatgctaagctcaggagcttgaccttcatcctaaaataaaaggcagcccaaaaagtttctggagagtgactgagctgggctttatgattatcttgatggactgaacacagggaggtcagggtagttgagcattaatgggaccctaaataagggtaaaaatggaaaaaagcaaaagaagactcatttcaaagagaactgacaggacacaagcaaattaggatgttggggctagtggtggtgtgtgaagaacaaggaatcaagtggaggggctgtcatgaacagaggtaggtaacaggaggaagagagcagtggccaaatctcatgttatctataccttcctttctctggcatc

SEQ ID NO: 15741 - RNA, 436 nt, Homo sapiens
  source 1..436: mol_type = other RNA
gctgggattacaggcatgagccactgtgcctggcagaggactgcatttttcgggagtttgtgtgttccatgtgtactccttgcactcacagcactgaaagtagtaagaagccacctggaagttttctggaaaaaaagccagtgcaggtttataaggaaagcagaggtgtggggcttgggaaaagcttttaattaaaaaatatgagttctaggcccagggctggcagtatctaactatgtaaccttgggtaagtcaccccctttcactcaaccttactttctacaccattaaaatgagggaataggaatgcaggggagtacaaattatccaacccatttactctgcctacagcagccagacgtttttttttcctggaggccaggcacggtggctcatgcctgtaatcccaacattttggaatgccaaggcaggagga

SEQ ID NO: 15742 - RNA, 215 nt, Homo sapiens
  source 1..215: mol_type = other RNA
gctgggattacaggcatgagccactgtgcctggcagaggactgcatttttcgggagtttgtgtgttccatgtgtactccttgcactcacagcactgaaagtagtaagaagccacctggaagttttctggcaggtcctgatggcacaatgagcaggtcattaccatggcctccatctgtccactcttagggcagtgtttctggccagctagtggca

SEQ ID NO: 15743 - RNA, 215 nt, Homo sapiens
  source 1..215: mol_type = other RNA
gctgggattacaggcatgagccactgtgcctggcagaggactgcatttttcgggagtttgtgtgttccatgtgtactccttgcactcacagcactgaaagtagtaagaagccacctggaagttttctttgctctggtccccatcattagcttttgaagatcttgcccagctggtctcctcagtacctgagaggtgacgcagacccatcttcctag

SEQ ID NO: 15744 - RNA, 1861 nt, Homo sapiens
  source 1..1861: mol_type = other RNA
gctgggattacaggcatgagccactgtgcctggccaaattaatttcttttgcatggttgctttcaccagtaagtggtccagaatacaaaatatggtaacagagaactgttttcatacttattccttggtacagttattaaaaataaaaactcgcattttaggattagggaagtctggaaaaaaatttttttaaacttggagatcacatattgaatagctgtcaaaattcaaactgactagttttgaagaacttcaaaaacgtgttcaaatgaataaagaacaaaaatgatcaaaagaaacccatagctgcctaagagtcttaaaaattattaatgtgacactctcatctctcatcaagtgtatccaaaccacttctcatttgctctttccatttaaagactcacagtagcttcactacacatatatttatactgaacatgtacagcggaacataaatatgatgagcatttatgaaaaaactactatctaagtggtttacactgacttgtgcgctgatctagtgagttaggagacctttttgatcttatcagtttcttgacatgctcagtgaaaaactgttgcacagaaactctaagtcccagctggtaatcaggcccatcgtccactggaggcaaagcttctgctgaatgagaagttgatttcagagttcttatattttccccaggcaccaaaaggcactactactgcagtactgttatcctcagtaccgtactgtattgcctgttcagtcaccgcatgggctgcttcgttgggatcatggcactgattgacaaagtcacaaatctcttgactattcaccatgaagttaattccatctgtggtgaggaccaggaagctgtcatcagcatgatgtaacttaatcctcttagtttcaggttctgctatgacaccactggtcttaaggtccaaatctccaatacttcttgtcattgcaagcctgccatttacgtgaggctgccccaaactattccaagctacaaaaccaccacatttcttgatcctttctttttcatcttttctttctggagtatggtcaatggtcagcttcatgggttttccttttctacacaaaatagcccggctgtccccaacactggctacaaccagttcaataccatctcgcaatagggctactgttgcagtagtcccagaggtcagaagagttgcatcagcagacaggcgggcatgactcgaaaaggctttatctatttctagaaaagccaaggtcaacagagtttccaagttcttctccttaggaagcaaatccataatacatttctccatgtgggtatgacagaaatcagctgctgcaggtccaccgtgtccatcatacactgcaaagtacaggacctcatctgtcagctgagcgaagtcaaaccgatcttcattctctttccgtttgccaatctgtgaggcgcaccccacattttccaagctgattttgggaattggcttgccatacttaatgctgggtggcagcagaattggctcatcaatgcggttatcccagatcccaaaattgtcccaggtagctggactcccactaccatctgggtcaaaccgagaacacctaggctctgaagtggagctgtggcacgtgggtgtcacccgcctgtcgtcctgcagcaggcgggagcttagcagcactctccttctcacctggttcccaccacttctgaccaaagtaattaaggcagctgttgacataactcagctccaaaggactcagtgatgagggaaaggtcaatggaacaataatggaatgtcccgacgagctgctcacgacctccaaagggaagaaagcgacgctctgagaactccgagaggccgccggccaagc

SEQ ID NO: 15745 - RNA, 1943 nt, Homo sapiens
  source 1..1943: mol_type = other RNA
gctgggattacaggcatgagccactgtgcctggccaaattaatttcttttgcatggttgctttcaccagtaagtggtccagaatacaaaatatggtaacagagaactgttttcatacttattccttggtacagttattaaaaataaaaactcgcattttaggattagggaagtctggaaaaaaatttttttaaacttggagatcacatattgaatagctgtcaaaattcaaactgactagttttgaagaacttcaaaaacgtgttcaaatgaataaagaacaaaaatgatcaaaagaaacccatagctgcctaagagtcttaaaaattattaatgtgacactctcatctctcatcaagtgtatccaaaccacttctcatttgctctttccatttaaagactcacagtagcttcactacacatatatttatactgaacatgtacagcggaacataaatatgatgagcatttatgaaaaaactactatctaagtggtttacactgacttgtgcgctgatctagtgagttaggagacctttttgatcttatcagtttcttgacatgctcagtgaaaaactgttgcacagaaactctaagtcccagctggtaatcaggcccatcgtccactggaggcaaagcttctgctgaatgagaagttgatttcagagttcttatattttccccaggcaccaaaaggcactactactgcagtactgttatcctcagtaccgtactgtattgcctgttcagtcaccgcatgggctgcttcgttgggatcatggcactgattgacaaagtcacaaatctcttgactattcaccatgaagttaattccatctgtggtgaggaccaggaagctgtcatcagcatgatgtaacttaatcctcttagtttcaggttctgctatgacaccactggtcttaaggtccaaatctccaatacttcttgtcattgcaagcctgccatttacgtgaggctgccccaaactattccaagctacaaaaccaccacatttcttgatcctttctttttcatcttttctttctggagtatggtcaatggtcagcttcatgggttttccttttctacacaaaatagcccggctgtccccaacactggctacaaccagttcaataccatctcgcaatagggctactgttgcagtagtcccagaggtcagaagagttgcatcagcagacaggcgggcatgactcgaaaaggctttatctatttctagaaaagccaaggtcaacagagtttccaagttcttctccttaggaagcaaatccataatacatttctccatgtgggtatgacagaaatcagctgctgcaggtccaccgtgtccatcatacactgcaaagtacaggacctcatctgtcagctgagcgaagtcaaaccgatcttcattctctttccgtttgccaatctgtgaggcgcaccccacattttccaagctgattttgggaattggcttgccatacttaatgctgggtggcagcagaattggctcatcaatgcggttatcccagatcccaaaattgtcccaggtagctggactcccactaccatctgggtcaaaccgagaacacctaggctctgaagtggagctgtggcacgtgggtgtcacccgcctgtcgtcctgcagcaggcgggagcttagcagcactctccttctcacctggttcccaccacttctgaccaaagtaattaaggcagctgttgacataactcagctccaaaggactcagtgatgagggaaaggtcaatggaacaataatggaatgtctctggatggctacgtccctgaaaaatgttttaattagctaacggaggacgggggaggagctttcttggtcggtaaataagagtgccttctccgtcgtctcggatctccgaagcaagcagtcaaagcggccactgccttgcctgctggaaattctc

SEQ ID NO: 15746 - RNA, 2274 nt, Homo sapiens
  source 1..2274: mol_type = other RNA
gctgggattacaggcatgagccactgtgcctggccaaattaatttcttttgcatggttgctttcaccagtaagtggtccagaatacaaaatatggtaacagagaactgttttcatacttattccttggtacagttattaaaaataaaaactcgcattttaggattagggaagtctggaaaaaaatttttttaaacttggagatcacatattgaatagctgtcaaaattcaaactgactagttttgaagaacttcaaaaacgtgttcaaatgaataaagaacaaaaatgatcaaaagaaacccatagctgcctaagagtcttaaaaattattaatgtgacactctcatctctcatcaagtgtatccaaaccacttctcatttgctctttccatttaaagactcacagtagcttcactacacatatatttatactgaacatgtacagcggaacataaatatgatgagcatttatgaaaaaactactatctaagtggtttacactgacttgtgcgctgatctagtgagttaggagacctttttgatcttatcagtttcttgacatgctcagtgaaaaactgttgcacagaaactctaagtcccagctggtaatcaggcccatcgtccactggaggcaaagcttctgctgaatgagaagttgatttcagagttcttatattttccccaggcaccaaaaggcactactactgcagtactgttatcctcagtaccgtactgtattgcctgttcagtcaccgcatgggctgcttcgttgggatcatggcactgattgacaaagtcacaaatctcttgactattcaccatgaagttaattccatctgtggtgaggaccaggaagctgtcatcagcatgatgtaacttaatcctcttagtttcaggttctgctatgacaccactggtcttaaggtccaaatctccaatacttcttgtcattgcaagcctgccatttacgtgaggctgccccaaactattccaagctacaaaaccaccacatttcttgatcctttctttttcatcttttctttctggagtatggtcaatggtcagcttcatgggttttccttttctacacaaaatagcccggctgtccccaacactggctacaaccagttcaataccatctcgcaatagggctactgttgcagtagtcccagaggtcagaagagttgcatcagcagacaggcgggcatgactcgaaaaggctttatctatttctagaaaagccaaggtcaacagagtttccaagttcttctccttaggaagcaaatccataatacatttctccatgtgggtatgacagaaatcagctgctgcaggtccaccgtgtccatcatacactgcaaagtacaggacctcatctgtcagctgagcgaagtcaaaccgatcttcattctctttccgtttgccaatctgtgaggcgcaccccacattttccaagctgattttgggaattggcttgccatacttaatgctgggtggcagcagaattggctcatcaatgcggttatcccagatcccaaaattgtcccaggtagctggactcccactaccatctgggtcaaaccgagaacacctaggctctgaagtggagctgtggcacgtgggtgtcacccgcctgtcgtcctgcagcaggcgggagcttagcagcactctccttctcacctggttcccaccacttctgaccaaagtaattaaggcagctgttgacataactcagctccaaaggactcagtgatgagggaaaggtcaatggaacaataatggaatgtctgggtacagctcaggatcctggcctcggctcgctggccctgacaggcgggtggtcagggtgacacacggtgggaagaacacacgcccgcctgcctgcgaagcctcgcaaatagctgggctccctcggcaccttctgccgccaggtctccgcctcccaacctccctctgggcgtaccgagcccgttgtcgccacgtttccctcgcccgggaggcaacgcggcacccaccccgcagcatcctcgcttccggggcctcgggcaagggtctccagtcccagcccacccaccctgcccgcctcgcgccgcgctggccctccagcctgcggccacattcaaggccgagcgcagtctgggctggaaacccgccgcccggggcgcaggcagcccagctgggccccgcctcaccccgacgagctgctcacgacctccaaagggaagaaagcgacgctctgagaactccgagaggccgccggccaagcgccgactc

SEQ ID NO: 15747 - RNA, 1452 nt, Homo sapiens
  source 1..1452: mol_type = other RNA
gctgggattacaggcatgagccactgtgcctggccaaattaatttcttttgcatggttgctttcaccagtaagtggtccagaatacaaaatatggtaacagagaactgttttcatacttattccttggtacagttattaaaaataaaaactcgcattttaggattagggaagtctggaaaaaaatttttttaaacttggagatcacatattgaatagctgtcaaaattcaaactgactagttttgaagaacttcaaaaacgtgttcaaatgaataaagaacaaaaatgatcaaaagaaacccatagctgcctaagagtcttaaaaattattaatgtgacactctcatctctcatcaagtgtatccaaaccacttctcatttgctctttccatttaaagactcacagtagcttcactacacatatatttatactgaacatgtacagcggaacataaatatgatgagcatttatgaaaaaactactatctaagtggtttacactgacttgtgcgctgatctagtgagttaggagacctttttgatcttatcagtttcttgacatgctcagtgaaaaactgttgcacagaaactctaagtcccagctggtaatcaggcccatcgtccactggaggcaaagcttctgctgaatgagaagttgatttcagagttcttatattttccccaggcaccaaaaggcactactactgcagtactgttatcctcagtaccgtactgtattgcctgttcagtcaccgcatgggctgcttcgttgggatcatggcactgattgacaaagtcacaaatctcttgactattcaccatgaagttaattccatctgtggtgaggaccaggaagctgtcatcagcatgatgtaacttaatcctcttagtttcaggttctgctatgacaccactggtcttaaggtccaaatctccaatacttcttgtcattgcaagcctgccatttacgtgaggctgccccaaactattccaagctacaaaaccaccacatttcttgatcctttctttttcatcttttctttctggagtatggtcaatggtcagcttcatgggttttccttttctacacaaaatagcccggctgtccccaacactggctacaaccagttcaataccatctcgcaatagggctactgttgcagtagtcccagaggtcagaagagttgctgggacaaaattaagcagatctctctttccactgaagccccgcatatagtgtccacgggctccaggtctagagctgctgaccaggcacagttctctgccacaaataacacgcacagaggcaaatacgaatttcacccaggaattgtgctcaaacattacaaaccatcagcagacaggcgggcatgactcgaaaaggctttatctatttctagaaaagccaaggtcaacagagtttccaagttcttctccttaggaagcaaatcc

SEQ ID NO: 15748 - RNA, 2141 nt, Homo sapiens
  source 1..2141: mol_type = other RNA
gctgggattacaggcatgagccactgtgcctggccaaattaatttcttttgcatggttgctttcaccagtaagtggtccagaatacaaaatatggtaacagagaactgttttcatacttattccttggtacagttattaaaaataaaaactcgcattttaggattagggaagtctggaaaaaaatttttttaaacttggagatcacatattgaatagctgtcaaaattcaaactgactagttttgaagaacttcaaaaacgtgttcaaatgaataaagaacaaaaatgatcaaaagaaacccatagctgcctaagagtcttaaaaattattaatgtgacactctcatctctcatcaagtgtatccaaaccacttctcatttgctctttccatttaaagactcacagtagcttcactacacatatatttatactgaacatgtacagcggaacataaatatgatgagcatttatgaaaaaactactatctaagtggtttacactgacttgtgcgctgatctagtgagttaggagacctttttgatcttatcagtttcttgacatgctcagtgaaaaactgttgcacagaaactctaagtcccagctggtaatcaggcccatcgtccactggaggcaaagcttctgctgaatgagaagttgatttcagagttcttatattttccccaggcaccaaaaggcactactactgcagtactgttatcctcagtaccgtactgtattgcctgttcagtcaccgcatgggctgcttcgttgggatcatggcactgattgacaaagtcacaaatctcttgactattcaccatgaagttaattccatctgtggtgaggaccaggaagctgtcatcagcatgatgtaacttaatcctcttagtttcaggttctgctatgacaccactggtcttaaggtccaaatctccaatacttcttgtcattgcaagcctgccatttacgtgaggctgccccaaactattccaagctacaaaaccaccacatttcttgatcctttctttttcatcttttctttctggagtatggtcaatggtcagcttcatgggttttccttttctacacaaaatagcccggctgtccccaacactggctacaaccagttcaataccatctcgcaatagggctactgttgcagtagtcccagaggtcagaagagttgctgggacaaaattaagcagatctctctttccactgaagccccgcatatagtgtccacgggctccaggtctagagctgctgaccaggcacagttctctgccacaaataacacgcacagaggcaaatacgaatttcacccaggaattgtgctcaaacattacaaacctgcaacacaggggagagcagagaaagagcatcagcagacaggcgggcatgactcgaaaaggctttatctatttctagaaaagccaaggtcaacagagtttccaagttcttctccttaggaagcaaatccataatacatttctccatgtgggtatgacagaaatcagctgctgcaggtccaccgtgtccatcatacactgcaaagtacaggacctcatctgtcagctgagcgaagtcaaaccgatcttcattctctttccgtttgccaatctgtgaggcgcaccccacattttccaagctgattttgggaattggcttgccatacttaatgctgggtggcagcagaattggctcatcaatgcggttatcccagatcccaaaattgtcccaggtagctggactcccactaccatctgggtcaaaccgagaacacctaggctctgaagtggagctgtggcacgtgggtgtcacccgcctgtcgtcctgcagcaggcgggagcttagcagcactctccttctcacctggttcccaccacttctgaccaaagtaattaaggcagctgttgacataactcagctccaaaggactcagtgatgagggaaaggtcaatggaacaataatggaatgtctctggatggctacgtccctgaaaaatgttttaattagctaacggaggacgggggaggagctttcttggtcggtaaataagagtgccttctccgtcgtctcggatctccgaagcaagcagtcaaagcggccactgccttgcctgctggaaattctcgaaaa

SEQ ID NO: 15749 - RNA, 1746 nt, Homo sapiens
  source 1..1746: mol_type = other RNA
gctgggattacaggcatgagccactgtgcctggccaaattaatttcttttgcatggttgctttcaccagtaagtggtccagaatacaaaatatggtaacagagaactgttttcatacttattccttggtacagttattaaaaataaaaactcgcattttaggattagggaagtctggaaaaaaatttttttaaacttggagatcacatattgaatagctgtcaaaattcaaactgactagttttgaagaacttcaaaaacgtgttcaaatgaataaagaacaaaaatgatcaaaagaaacccatagctgcctaagagtcttaaaaattattaatgtgacactctcatctctcatcaagtgtatccaaaccacttctcatttgctctttccatttaaagactcacagtagcttcactacacatatatttatactgaacatgtacagcggaacataaatatgatgagcatttatgaaaaaactactatctaagtggtttacactgacttgtgcgctgatctagtgagttaggagacctttttgatcttatcagtttcttgacatgctcagtgaaaaactgttgcacagaaactctaagtcccagctggtaatcaggcccatcgtccactggaggcaaagcttctgctgaatgagaagttgatttcagagttcttatattttccccaggcaccaaaaggcactactactgcagtactgttatcctcagtaccgtactgtattgcctgttcagtcaccgcatgggctgcttcgttgggatcatggcactgattgacaaagtcacaaatctcttgactattcaccatgaagttaattccatctgtggtgaggaccaggaagctgtcatcagcatgatgtaacttaatcctcttagtttcaggttctgctatgacaccactggtcttaaggtccaaatctccaatacttcttgtcattgcaagcctgccatttacgtgaggctgccccaaactattccaagctacaaaaccaccacatttcttgatcctttctttttcatcttttctttctggagtatggtcaatggtcagcttcatgggttttccttttctacacaaaatagcccggctgtccccaacactggctacaaccagttcaataccatctcgcaatagggctactgttgcagtagtcccagaggtcagaagagttgctgggacaaaattaagcagatctctctttccactgaagccccgcatatagtgtccacgggctccaggtctagagctgctgaccaggcacagttctctgccacaaataacacgcacagaggcaaatacgaatttcacccaggaattgtgctcaaacattacaaacctgcaacacaggggagagcagagaaagagcatcagcagacaggcgggcatgactcgaaaaggctttatctatttctagaaaagccaaggtcaacagagtttccaagttcttctccttaggaagcaaatccctctggatggctacgtccctgaaaaatgttttaattagctaacggaggacgggggaggagctttcttggtcggtaaataagagtgccttctccgtcgtctcggatctccgaagcaagcagtcaaagcggccactgccttgcctgctggaaattctcgaaaatttttctcccgcagttgaccagatggagagggagaagtctgttcccgctgactgacagcagatccggccagtccgcactcggcgagacggctggccggccgccc

SEQ ID NO: 15750 - RNA, 2141 nt, Homo sapiens
  source 1..2141: mol_type = other RNA
gctgggattacaggcatgagccactgtgcctggccaaattaatttcttttgcatggttgctttcaccagtaagtggtccagaatacaaaatatggtaacagagaactgttttcatacttattccttggtacagttattaaaaataaaaactcgcattttaggattagggaagtctggaaaaaaatttttttaaacttggagatcacatattgaatagctgtcaaaattcaaactgactagttttgaagaacttcaaaaacgtgttcaaatgaataaagaacaaaaatgatcaaaagaaacccatagctgcctaagagtcttaaaaattattaatgtgacactctcatctctcatcaagtgtatccaaaccacttctcatttgctctttccatttaaagactcacagtagcttcactacacatatatttatactgaacatgtacagcggaacataaatatgatgagcatttatgaaaaaactactatctaagtggtttacactgacttgtgcgctgatctagtgagttaggagacctttttgatcttatcagtttcttgacatgctcagtgaaaaactgttgcacagaaactctaagtcccagctggtaatcaggcccatcgtccactggaggcaaagcttctgctgaatgagaagttgatttcagagttcttatattttccccaggcaccaaaaggcactactactgcagtactgttatcctcagtaccgtactgtattgcctgttcagtcaccgcatgggctgcttcgttgggatcatggcactgattgacaaagtcacaaatctcttgactattcaccatgaagttaattccatctgtggtgaggaccaggaagctgtcatcagcatgatgtaacttaatcctcttagtttcaggttctgctatgacaccactggtcttaaggtccaaatctccaatacttcttgtcattgcaagcctgccatttacgtgaggctgccccaaactattccaagctacaaaaccaccacatttcttgatcctttctttttcatcttttctttctggagtatggtcaatggtcagcttcatgggttttccttttctacacaaaatagcccggctgtccccaacactggctacaaccagttcaataccatctcgcaatagggctactgttgcagtagtcccagaggtcagaagagttgctgggacaaaattaagcagatctctctttccactgaagccccgcatatagtgtccacgggctccaggtctagagctgctgaccaggcacagttctctgccacaaataacacgcacagaggcaaatacgaatttcacccaggaattgtgctcaaacattacaaacctgccaggttctatgcagggtgctgcacacatcagcagacaggcgggcatgactcgaaaaggctttatctatttctagaaaagccaaggtcaacagagtttccaagttcttctccttaggaagcaaatccataatacatttctccatgtgggtatgacagaaatcagctgctgcaggtccaccgtgtccatcatacactgcaaagtacaggacctcatctgtcagctgagcgaagtcaaaccgatcttcattctctttccgtttgccaatctgtgaggcgcaccccacattttccaagctgattttgggaattggcttgccatacttaatgctgggtggcagcagaattggctcatcaatgcggttatcccagatcccaaaattgtcccaggtagctggactcccactaccatctgggtcaaaccgagaacacctaggctctgaagtggagctgtggcacgtgggtgtcacccgcctgtcgtcctgcagcaggcgggagcttagcagcactctccttctcacctggttcccaccacttctgaccaaagtaattaaggcagctgttgacataactcagctccaaaggactcagtgatgagggaaaggtcaatggaacaataatggaatgtctctggatggctacgtccctgaaaaatgttttaattagctaacggaggacgggggaggagctttcttggtcggtaaataagagtgccttctccgtcgtctcggatctccgaagcaagcagtcaaagcggccactgccttgcctgctggaaattctcgaaaa

SEQ ID NO: 15751 - RNA, 91 nt, Homo sapiens
  source 1..91: mol_type = other RNA
gctgggattacaggcatgagccactgtgcctggccaagatttgttgtttaatgttgacttttggtcaggcacagtcgctcatgtctgtaat

SEQ ID NO: 15752 - RNA, 3898 nt, Homo sapiens
  source 1..3898: mol_type = other RNA
gctgggattacaggcatgagccactgtgcctggccagctctgcctttttatgatactgaagatctaggcttcatttggaatttcctcaccttcctgtggacaaaattcctcctttgattgtgtcccagccacatctagttgcttcggtaggtaatcttaatgtgcagttctacttgtcctttatgctatattgcaaactccaaagatataatcacactagtatttatgtgtttaagtgtgtgtatgttaaacatgtaaaggggtaatgtatctatacagatatatgtatacttcccatttaagcaaaagttaatttggttttacagatacagataccaggttctggcagcttggagaataagtgtaacaatttggtaaaacttgtataattctgactgacctataatattacagagtgaatttcaagttattgctttttgattacagaataaaaaattcattctcttgcaaaacttttatacagaatgagtaaccatttcctattcaagtaacagcaatcagaatcagaagttccttacacaacagtagatgcttgagacattttttgaatggagatgtgatttcattctgttcaagaacttatgcaggaaactgggagtgacttaatttttcaaaagtacaagaaaatcagcaccccaactgcttagtgctcaggagggtttctcaagggctctataaagctcagcttgtggtgagttcacacccacctttagaaggattcccattctacttatgcagccttgtttcagaacacaaagcttgtattaaaacattaaaagaggattaaaagcagtgttggtttttaacattcagaattcacagaggatctcattttctgtaattaaatgatctattttgtgttttttgctgcagaatcacattcatatggcagtcatatttcaggcacttttaaaacatgttcatctggaataaaaatctgcatgaaccacttctgcataattcaaaatgagtgttgagtgattctagttctcaaatagatagcaaatcaccacctggtgattcgctttcttcatcacaacatgacggtgactgctgagcttgagacatctttgaggtgcctttctggcttcagtaaaaagatgtgagccataaaaatccaaactactcagtttctacttaaaaaaatacaaaatggtgaaatatactaaatgtattatacagatggtttcagctactatcaaaataaataacataatctgactcagaagtctgactgagcttttggacgaaatctgatggaatgtcaaacgtggagactccctcctagggactagctgctggtaggcaaaagtaactcaacatccttaccatttgctacaacagtattggaagagcagctgctggcaaggtcttctgcagtggtcaaagaggctgcctgggaatgagttttggtcaatggagtggtagcagatggagaaggggtgaggccaggtttcttgggtgggatgggtggagggtttcctctctcagctctggggatggttggggacttgattcctggagacagggggctcaggggactggacactttccctggagtaggtgaatggcttgtgtcacctcttggattggcagtgttggctagatttcgatagtctgtgccaaagggagagctgttgggagagactggcttgattggcccttgttggctagtgaatctggagagcacctgagtgactgtgtttcgggccagctgcttggcggcagagttgtctatgagggtgggggataaatccctggatggagggctctgtaggccactggcttgttggtcctgatctgcttgggactgaaatttgtggcgagctgcatggaaccgttggttgatccctacttggtacgatgactggtagccagggctgctagctgatgaccccaataaacgcttagtgagtaccggcgaagagcaaggagaggatgttagagaggaggaggcagtgctgctgggagacagtgagctcccactggaagagaggggactgggcattgggactggagtctcaatccccacaggacacccaccattctccactggtttctcttgggccaatgccacagatttttcccgtggaggcacctggttttctacattgttgcctgcagtcagctccctggtagtttgtatctctgggtcacaatggccattggtttttgcatatgagtaagcaggagtggcaggaccaggcagcccagtgtttgtcatcttggctatgttgctcccatgggttctttctgctggaaaactctctgtttggcaaaacacagacattagcatgagaggctcagttgctgtgcctttggacacggttactggtttcttcaattgctcattagggctactgtgctggtgggaagcctctaggtccttcactatcttctttaaactttccatttcttctttcagggttttggtccggttctcttctcggttcagttttgctctcagttgttccctttcgatgtcaaactctgataactgcttctctacctgggcctcagtctgcaagcctctctttctctcagctgccaactcttcttccagtttactcacccggctcttctccttctccaatttcaggctcagctctcctgccttctgtccttcctcggctgccttgttggtggctttcttgcactcaagcactagcatggatgagagctgcttgtggcgggagcgctcctcttccagctgactagagagcttcttctgttctttttcaaactttttcacttgggatttttcaaattccaactgttgagtcagcctctctctttccttctctagcatgtaggtgacatcatctccttcagccgtatcctgtgcatgccgctgcctttcttcctcaaggtctaggatcacctttcggtgcctgctctcagcagcagccagctgggacagcatgcgctcctgcatgttcttgcactgcttcatcacaaccttaagaatagagagtggatttgtgcagactggctgcttttcgccatcatttttctccttcagtgtttcaaaatctctctgtagagccattaaaggatcactgatgttatattttccatagcgttcttcaatgaaagtatctctgtgttgggcctttaaggcttctataacaaggtcccttgcttcaagctctccttcaagaatactaaatagtgtcaggagttcaggcttgctgagtttttccagattcatcttgaaagcctgataatcggcagagtcacacttcagtcctcaagtataaacttacagttttcttcagtaaaaaattgggaaaattgccaaatatatttaaaatgccattagcatggtggaaatgtgtccaatgctgaacttgtttcctcatttgttaaatgagataatagctcctgtctacaagaccaggtggttgtcagtatccaagcgatctgatgtacatggaagtattagctacctgggagatcttgctcaatcctcttctctgagtcctaggctccaactaaacatctgggactccataaggctccttctagctgtggcccactggactgggacttattaagatgctgagtgctgagtgagctagatgtagaagttgaaatgaatgggaaaagtgatgaaaagaaatgctttctttcttctggcttgtcttcactatctccttttcctcacgcttcccgaccccaccccttctccccggggttgatgaggaggtcaaagtctgaaagccagagagggctctccaagccccggaccaggctgaagccgaaggcaaggtgtgccctccactgccccctgcatttctgcattttctcccatcatttgttcccacaaaggatttgctgggcagtccttaaacgttctcttcttgcttggatctgc

SEQ ID NO: 15753 - RNA, 3531 nt, Homo sapiens
  source 1..3531: mol_type = other RNA
gctgggattacaggcatgagccactgtgcctggccagctctgcctttttatgatactgaagatctaggcttcatttggaatttcctcaccttcctgtggacaaaattcctcctttgattgtgtcccagccacatctagttgcttcggtaggtaatcttaatgtgcagttctacttgtcctttatgctatattgcaaactccaaagatataatcacactagtatttatgtgtttaagtgtgtgtatgttaaacatgtaaaggggtaatgtatctatacagatatatgtatacttcccatttaagcaaaagttaatttggttttacagatacagataccaggttctggcagcttggagaataagtgtaacaatttggtaaaacttgtataattctgactgacctataatattacagagtgaatttcaagttattgctttttgattacagaataaaaaattcattctcttgcaaaacttttatacagaatgagtaaccatttcctattcaagtaacagcaatcagaatcagaagttccttacacaacagtagatgcttgagacattttttgaatggagatgtgatttcattctgttcaagaacttatgcaggaaactgggagtgacttaatttttcaaaagtacaagaaaatcagcaccccaactgcttagtgctcaggagggtttctcaagggctctataaagctcagcttgtggtgagttcacacccacctttagaaggattcccattctacttatgcagccttgtttcagaacacaaagcttgtattaaaacattaaaagaggattaaaagcagtgttggtttttaacattcagaattcacagaggatctcattttctgtaattaaatgatctattttgtgttttttgctgcagaatcacattcatatggcagtcatatttcaggcacttttaaaacatgttcatctggaataaaaatctgcatgaaccacttctgcataattcaaaatgagtgttgagtgattctagttctcaaatagatagcaaatcaccacctggtgattcgctttcttcatcacaacatgacggtgactgctgagcttgagacatctttgaggtgcctttctggcttcagtaaaaagatgtgagccataaaaatccaaactactcagtttctacttaaaaaaatacaaaatggtgaaatatactaaatgtattatacagatggtttcagctactatcaaaataaataacataatctgactcagaagtctgactgagcttttggacgaaatctgatggaatgtcaaacgtggagactccctcctagggactagctgctggtaggcaaaagtaactcaacatccttaccatttgctacaacagtattggaagagcagctgctggcaaggtcttctgcagtggtcaaagaggctgcctgggaatgagttttggtcaatggagtggtagcagatggagaaggggtgaggccaggtttcttgggtgggatgggtggagggtttcctctctcagctctggggatggttggggacttgattcctggagacagggggctcaggggactggacactttccctggagtaggtgaatggcttgtgtcacctcttggattggcagtgttggctagatttcgatagtctgtgccaaagggagagctgttgggagagactggcttgattggcccttgttggctagtgaatctggagagcacctgagtgactgtgtttcgggccagctgcttggcggcagagttgtctatgagggtgggggataaatccctggatggagggctctgtaggccactggcttgttggtcctgatctgcttgggactgaaatttgtggcgagctgcatggaaccgttggttgatccctacttggtacgatgactggtagccagggctgctagctgatgaccccaataaacgcttagtgagtaccggcgaagagcaaggagaggatgttagagaggaggaggcagtgctgctgggagacagtgagctcccactggaagagaggggactgggcattgggactggagtctcaatccccacaggacacccaccattctccactggtttctcttgggccaatgccacagatttttcccgtggaggcacctggttttctacattgttgcctgcagtcagctccctggtagtttgtatctctgggtcacaatggccattggtttttgcatatgagtaagcaggagtggcaggaccaggcagcccagtgtttgtcatcttggctatgttgctcccatgggttctttctgctggaaaactctctgtttggcaaaacacagacattagcatgagaggctcagttgctgtgcctttggacacggttactggtttcttcaattgctcattagggctactgtgctggtgggaagcctctaggtccttcactatcttctttaaactttccatttcttctttcagggttttggtccggttctcttctcggttcagttttgctctcagttgttccctttcgatgtcaaactctgataactgcttctctacctgggcctcagtctgcaagcctctctttctctcagctgccaactcttcttccagtttactcacccggctcttctccttctccaatttcaggctcagctctcctgccttctgtccttcctcggctgccttgttggtggctttcttgcactcaagcactagcatggatgagagctgcttgtggcgggagcgctcctcttccagctgactagagagcttcttctgttctttttcaaactttttcacttgggatttttcaaattccaactgttgagtcagcctctctctttccttctctagcatgtaggtgacatcatctccttcagccgtatcctgtgcatgccgctgcctttcttcctcaaggtctaggatcacctttcggtgcctgctctcagcagcagccagctgggacagcatgcgctcctgcatgttcttgcactgcttcatcacaaccttaagaatagagagtggatttgtgcagactggctgcttttcgccatcatttttctccttcagtgtttcaaaatctctctgtagagccattaaaggatcactgatgttatattttccatagcgttcttcaatgaaagtatctctgtgttgggcctttaaggcttctataacaaggtcccttgcttcaagctctccttcaagaatactaaatagtgtcaggagttcaggcttgctgagtttttccagattcatcttgaaagcctgataatcggcagagtcacacttcagtcctcaagtataaacttacagttttcttcagtaaaaaattgggaaaattgccaaatatatttaaaatgccattagcatggtggaaatgtgtccaatgctgtgagtcctctccgccaaggctgaggtgcggggtgggaggtgcctttgaatgaggggtgtcagagggaagccccttctgaggagctgggaatcgacgagggacaaaaagtagctgtgaggaccctcggaggatgaggagccgcctcctcggggaataccgggag

SEQ ID NO: 15754 - RNA, 3424 nt, Homo sapiens
  source 1..3424: mol_type = other RNA
gctgggattacaggcatgagccactgtgcctggccagctctgcctttttatgatactgaagatctaggcttcatttggaatttcctcaccttcctgtggacaaaattcctcctttgattgtgtcccagccacatctagttgcttcggtaggtaatcttaatgtgcagttctacttgtcctttatgctatattgcaaactccaaagatataatcacactagtatttatgtgtttaagtgtgtgtatgttaaacatgtaaaggggtaatgtatctatacagatatatgtatacttcccatttaagcaaaagttaatttggttttacagatacagataccaggttctggcagcttggagaataagtgtaacaatttggtaaaacttgtataattctgactgacctataatattacagagtgaatttcaagttattgctttttgattacagaataaaaaattcattctcttgcaaaacttttatacagaatgagtaaccatttcctattcaagtaacagcaatcagaatcagaagttccttacacaacagtagatgcttgagacattttttgaatggagatgtgatttcattctgttcaagaacttatgcaggaaactgggagtgacttaatttttcaaaagtacaagaaaatcagcaccccaactgcttagtgctcaggagggtttctcaagggctctataaagctcagcttgtggtgagttcacacccacctttagaaggattcccattctacttatgcagccttgtttcagaacacaaagcttgtattaaaacattaaaagaggattaaaagcagtgttggtttttaacattcagaattcacagaggatctcattttctgtaattaaatgatctattttgtgttttttgctgcagaatcacattcatatggcagtcatatttcaggcacttttaaaacatgttcatctggaataaaaatctgcatgaaccacttctgcataattcaaaatgagtgttgagtgattctagttctcaaatagatagcaaatcaccacctggtgattcgctttcttcatcacaacatgacggtgactgctgagcttgagacatctttgaggtgcctttctggcttcagtaaaaagatgtgagccataaaaatccaaactactcagtttctacttaaaaaaatacaaaatggtgaaatatactaaatgtattatacagatggtttcagctactatcaaaataaataacataatctgactcagaagtctgactgagcttttggacgaaatctgatggaatgtcaaacgtggagactccctcctagggactagctgctggtaggcaaaagtaactcaacatccttaccatttgctacaacagtattggaagagcagctgctggcaaggtcttctgcagtggtcaaagaggctgcctgggaatgagttttggtcaatggagtggtagcagatggagaaggggtgaggccaggtttcttgggtgggatgggtggagggtttcctctctcagctctggggatggttggggacttgattcctggagacagggggctcaggggactggacactttccctggagtaggtgaatggcttgtgtcacctcttggattggcagtgttggctagatttcgatagtctgtgccaaagggagagctgttgggagagactggcttgattggcccttgttggctagtgaatctggagagcacctgagtgactgtgtttcgggccagctgcttggcggcagagttgtctatgagggtgggggataaatccctggatggagggctctgtaggccactggcttgttggtcctgatctgcttgggactgaaatttgtggcgagctgcatggaaccgttggttgatccctacttggtacgatgactggtagccagggctgctagctgatgaccccaataaacgcttagtgagtaccggcgaagagcaaggagaggatgttagagaggaggaggcagtgctgctgggagacagtgagctcccactggaagagaggggactgggcattgggactggagtctcaatccccacaggacacccaccattctccactggtttctcttgggccaatgccacagatttttcccgtggaggcacctggttttctacattgttgcctgcagtcagctccctggtagtttgtatctctgggtcacaatggccattggtttttgcatatgagtaagcaggagtggcaggaccaggcagcccagtgtttgtcatcttggctatgttgctcccatgggttctttctgctggaaaactctctgtttggcaaaacacagacattagcatgagaggctcagttgctgtgcctttggacacggttactggtttcttcaattgctcattagggctactgtgctggtgggaagcctctaggtccttcactatcttctttaaactttccatttcttctttcagggttttggtccggttctcttctcggttcagttttgctctcagttgttccctttcgatgtcaaactctgataactgcttctctacctgggcctcagtctgcaagcctctctttctctcagctgccaactcttcttccagtttactcacccggctcttctccttctccaatttcaggctcagctctcctgccttctgtccttcctcggctgccttgttggtggctttcttgcactcaagcactagcatggatgagagctgcttgtggcgggagcgctcctcttccagctgactagagagcttcttctgttctttttcaaactttttcacttgggatttttcaaattccaactgttgagtcagcctctctctttccttctctagcatgtaggtgacatcatctccttcagccgtatcctgtgcatgccgctgcctttcttcctcaaggtctaggatcacctttcggtgcctgctctcagcagcagccagctgggacagcatgcgctcctgcatgttcttgcactgcttcatcacaaccttaagaatagagagtggatttgtgcagactggctgcttttcgccatcatttttctccttcagtgtttcaaaatctctctgtagagccattaaaggatcactgatgttatattttccatagcgttcttcaatgaaagtatctctgtgttgggcctttaaggcttctataacaaggtcccttgcttcaagctctccttcaagaatactaaatagtgtcaggagttcaggcttgctgagtttttccagattcatcttgaaagcctgataatcggcagagtcacacttcagtcctcaagtataaacttacagttttcttcagtaaaaaattgggaaaattgccaaatatatttaaaatgccattagcatggtggaaatgtgtccaatgctttccacgacgctccgggctccgctcccctccgcctccactccccatccacagcggct

SEQ ID NO: 15755 - RNA, 2467 nt, Homo sapiens
  source 1..2467: mol_type = other RNA
gctgggattacaggcatgagccactgtgcctggccaggactgtgatgttaaaagtttgctaaagaaataatcaagaacaaaaccaggttagattgagacaaaaaacaagctagcagtgagtgagctgtatagtgcctgctgacttaggtggcgtgtttcagcttggcacactgataaatccattgagcaatcaatagatactctttttgatgaagttaaaaaagaaagtgagaaagaaacaccttcattacaaataggagatctagggccacaagagtccttgaagacgtttaacaacacaaacagtccacaccattgataagagaataaataagaataaaacctaagttgctaatatactggaaatatcaggaaaaaggaaataacaaatgaacttagggagaagcagagcattgtaggacagataaggctcagagaagaatgctaagttaaatgaaaacataagactaggacagaacttaagttaaagacatgctttttaaaatagacaagtcactggaggacacactaaaatgactgacccaaatcggatttaaatgagatgtgccattccatggtttacttttaaatagagtaaatattaattatattttggccatctttgaaacttatctccccaactgcatatacaaggtataactataaagtaatgagacttaagaaaccaccagctacaaacacaccagacctttttatcagatgagtgtggtcctttgatattatcacatcaggtacaataacagtaaaatctgtattattatagtaatttatattttgaacaacactttaatatccattttccttattccaacttatcttcaacaaccccatatgacagatattttaaagatgaggctcagagaagtatcttgttaaatgtgacacacttaaaagtgaagcaggactagactgactccttgctttgtgttcttttcagcacaacttgttgccttaccatataattaatccagagatgctgccattactcaaaacgtttttggaactcctcttttggaagtgcctccagagccacttatttatcagtcttgactccgaatgacttttggctgtccaaaaatcaaatccaccctcaaaggacgaagatttcccatcattgaggataatcaaaagaatgtgtcgcagactctttattgttatagacatctaggtaattgggggcagagaaaattgtaataagtgatggaaagcctgtggcttggctcttcctgtacattcgatacccagcatcttgggcttcatgggctctgataattgatagtaaattattgttctgcaaaaattcacaaactgcagggtaactgtagaaataagagcaccctcggacagtgttgtgggtatagtgctccaaggtcttctcattgccataatcctctgagggatcagaccaaagcaggtcacacacaggtccaaaggcgggaggttccgtaaacctgtctaatttcctaatgtcatctaaagaagtaatttcaggtgacattcctccatgtacacagagaaactgctggtttaagagggcagcaagaggaagacagtcaaatgtctccatacaggcatcatacacctgttccgaatatttgattcgacattcctgtttgaaggtgaaatagtctgtaagatgcctgcattcatgatttccccgaagcagaaacaatgttttgggatgattaatctttaaactccataaatacagcacacactctatactgaaatagcctctgtccacatagtcacccagaaagaggtagcgtgtgttactaggtgatcctccaacttcaaataacttcattaggtcaaagaattgtccatgaatatcaccacatactgtgattggagcatctacttctatcatagtcttctcttgcctcaggatggcagccccatcattgattatctttaaggctacttcctcttccagtcgtccttcctttaccaaatggttttttaaaacatcaactttaggtttcccattctcaaatacttccttgaaagtaagccgttgggttggaggaaaggggacagctttgatgacgcggtcggtggtggagaggtggaagcgcctcccggacatggtcccctcggcctcctccaggctccaggagcccgccggacgtgcgcctacgccgcggccgccgccttctcctcgggcagccttagctgcccggagccgtcagccagccgtgcccggccccggctcctcagcggtgtccgagcaccagaagggcgcggccaccgcagcgccggcctccgacgccactgacaggacgagggcccaccggccgctctcttgggaggcgccagcggctaaggcggggaacaccgcttcggcaccgaccgcgaccgctgctaagggtggcgaccgggacggccgcggctgctcgcggcccgggccctcgtgcacgcaagcgcgcccccgagcgccgctctc

SEQ ID NO: 15756 - RNA, 6124 nt, Homo sapiens
  source 1..6124: mol_type = other RNA
gctgggattacaggcatgagccactgtgcctggccaggatcatgtttctttaaaccacacatgatacccagaaggcatcataatagagttggcttcatcatcttccttatcataggttatgcttgatttcaaaagaaatttgttcctcgacaatacacagaaaatgcacttaacaatagcccctgaagttttccccagccaatgactggttagcagtctaataaggatcatattggacaagtatctttaacacaaaacagcacagggaatcatgggccactctcatcgttaggctctcttcacaggtatagcctatgttagaaggcttctgaaccacagatgctaaagaaaaattagttaaactgaagactgatgaagtattccctacaaatgaaaaggcaatcttatatgacaaaggacactatcaggaggttgaaaaacaacctatagaatgggagaaaatatttgtaaatcatatgtctatgattaatatccagaatatataaagaactcctgtaagtcaacaaccatcaccacacccagttcacaaatgggcagaggaatcttatggacatttctccagcggagatatatgcacagccaaggagcacgtgaaaagatactcagcatcattagttgctagagaaatgcaaagcaaaccccaagaaggtaccacttcctagccagcaggatgtagctattaaaacaacaacagaaaatcagtgttggcaagggtgtggaggaattgcagtccgtgtgcgttgctggtgggaatgtaaaatggcatagtcattgtggaaaggagtgtggcagttcctccaagagtcgcatatagaattgtcacatggtccagcaattccattcctaggttacccaaaagaatggaaagcaggggagctggaggccattatgctaagtgaagtaactcaggaagggaaagccacattcctatgttctcaggtataagtgggagctaagctgagggtccacaaaggcagagtggaggaatggacattggagactccgaaggggaaaggagatggaggattaaaacgctacattttgggtacaacatatactacttcggtgacaggtgcaccacaatctcagacctcaccactatacagttcatccacgtaaccaaaaaccacttggacccctaaagctattaaataaaataaataaatataaacattcagtaacattatctttagaagaacactttttaataaacctgggcatgaagaaaaaaggctgaataatattccatcgtatgcgtgtgtatatccatatatatatatatatatatatatatgcacacacacacacaatgtatatgtctagtgttaccaacttagtttcctttccttcaatattaaacgtctcatatttcccccagactttttgagagatagttgagaaataaagctgtgtaagtttagagtgtagtatgtgatgatttgatatatattgtgaaattattaacacaagttaggtgacacacctgtcacctgtcctagttatcattttttttttgtattgtagtgaaataaatgtctcatttaaaaaaaaagaattgaaagcaggaaatgaaacagatacttgaataccaatgctcatagtagcattaagcataatagccaagaggtaggaacaacccaattgttcatccacaaatgaggagagaaaatgtggtatgtaaatataatggaatatacgtttcatggaaaagaatgtatctttcaatttttaatttttgtgggtacatagtaggtgaatatatctatgggatccatgagatgttgggatacagacatgcaatgtgaaataagcacgtcatggagaatggggtatccatcccctcaagcatttatcctttgagttacaaacaattcaattacactcttttaggtacttaaaaacgtacaattaagttgttatagtcaccctgttgtactttcaaatactagatcttattctttcaaaaattggttgaacctattaaccatccccacatcccccatactctcccaatacctttcccagcctctggtaaccatccttctactctctatgcccatgagttcaattgctttgatttttaggtctcacaaacaagtgagaacatgtgatgtttgtctttctgttcctggcttatttcacaaaatgatctccatttccatccatgatgttgcaaacaacaggatctcattcttttccatggctgaatagtactccattgtgtatatataccacattttctttatccattcacctgttgatggacatttaggttgcttccaaatctaatggaatatattattcactcataaaaagtgtgaaattctgatacatgctgttaatataacacggatgtaccttgcaagcatgttgagtaacataagccacaccccaaaggacaaatattgtatgattccacttatacaaggtacctggcacaggcaaattcatagagacacaaagtagaatggtggttaccgggggccgggggagtagggagtggggagttgttacttaatgggtagagtttgtttgtttgggaaggttctggagataaaggatgtgatggttgcacaacaatgtgaacgggcgcaatgccactaaactgtgcgcttagttgcaaggttacaataggacattttatgtatatttcaccacaataaaaataggaaaaggcaggtgatttctaaggacacaagtcccttggggttgctagttctgtcagacttttccccttgtttttctgaatgacaaggattagtagtggataataatgagtggattcatggatttgagcaggacatgaaagaatttccatagacagagatgaaagggcatttctgacttgaaacctgggatgagcaccgatgcaggagaggcacgaaagctcacagcgtgttcagggcgtagtgaatagaggggtgcgtgccccgagcctgcagagcgggcagggatgtgtaggaaggcaccttcatcctcctcactcagcctcccagctccaggtccaaagccgccaaatcatctttcttgtcaccatcacatgataagggggagtccttccagactgccagtcaatgaagtaacacacacagccacggtcatgccagtctgagcccatcgggcgagccctgaggggaataacagtcttggtggcattgggcaagccccgaggactccatctcggggaataacagtcttggtggcatcggcgcttcaccaggcctcctggaaccatattcgggatccccaactgagtgctggaaagaccactggtcaggagcagggagcaggggtggaaggaggtggctcgtcctgaccttgacaatgagaatcctgttttaagcttcacgctgctgactaaacagaaaggccacggcacagggacagacgtgcgcatgaaatcacaggaagaaagacatttcacgaacaaatgcatcctcccaaaccagtctgaatccctccggacagggtgatgttaccacgcaactggcctggcctaatgagctggtttctgtcatccctcctggaaggttaccctgaaacactcactcacactcatggaaaagcacaggaatgttctaaaaatgcaagtttatcacgaaggagacacaggaggttcagagacgatgaagcggcaagccgggaggaaagatctgagagaagccaccaggctggggcagcatttcattatatccagaattccacttgggctctgcagtttctttcttcctgagaattatttaaaagtcccctccactgcgcatattgaagacagagcccaagacgcatccaggtgcaacgtctctgctaagaatgtgtgccaggaatggggcctggcttcctcgtcgagtgcggctgtccgtgggtttctgctagacagataacgttctgaaggagttaaactttcacagctcctcctcctcctcctcctcctctatatcccttacctcgccacgttcatcactggtcattttgctggaagggaagccctggtatattcttacattgctctggaagtgagctttagcccagcgtcgccaaacttacaccttaattgatcccagatgagaaggaaaagctattgctcttaccccacagtcttccctccctgaggccagaagcaggtcacgtgtaaaatggtctgctctctgctgacagtggcctgagtctcccatagtgtctgctgagctggatagtccctctccagggagctttgcaggggatgggtgatgagacatggacatggggacgaattcctctcatctggaatcgcagacacagcatggagatatgagcacgcggcatgggaaataggcttcctcagcccttcaggatcagggaacgtgccagagatgcaatgacatttggcagcagttgagagtatgagtgctcagcagcagcatctgcagactcgtgtggggacttctgtctggactcagggatgttaagagtagaaggcccaatgtcagcttctcacgtgggctgtcagcaccgcagatgataccggaagatggactgtgatgggccagcgacccctctgactgcacgcagctgtcagccaggcctggaacaggaggggcgagggggtgggctcagcctctgttagtgggagaggtcctggttggaagtttcactgaagtatcagtgttgactttctcaggtcaaatctgggccatttcatgcggtaaatccatgtcggcaggtatcagcccaagtgttttgaacatgctgcacttgtacatgcctggaccaaatgccaggctgatgagcagggaggggttgaaaagcagaagggagcccaacccaccggcgtcagcaggaggctggccctggctgtggctccccgatcagacaggcggcgtccaatggggcaccacacgactcccgccagggtggggcttcccctgtacctttcttagagctgatggtcccctgaccccactcgcagcctggaaggaggggatccctggcagagaccgggcttggcagaaaactgggcatctgcttgagaggtggaaatgctggagcatgcagaaaatctaagaacccttatttatatggggccccagaccaggaccctcgggtcagtctttctttgcccagggatggcatagcagtaacatcgcttcctgtgccctttccagtaatgtgagggcaccatctccgcccctgaactcccttcaggccacttcactccatttcctcagcctgaccacattacccctgccccagtacttggcttccctcaccatcacctaagtgaagctcacatgcacctctggagggagacaggcgcggggagagggagcctcagctggaggtgcaggaactgagtatcaatccattcacgggattgaggttctggtacccaaattcagaattttacgaaaatccaagacacttgttcattcgtgtgcaggaaaaaggtattcctagcccccaaaccacacctaacctgacagtgggcactcacttcaccttgagagggatcgatgtggtgaggaagttcaaggttgctagatggcatggaaaggaggcaatgggaaggaagtagatacccgccaggatatttctgtgaagctgttgtagcccagtgaaatgtcactctccaggtgtttttaccttctctactcccagctcacacggtgccctggcacgggtattggcaggactctccaggtgtttttaccttctctactcccagctcacacggtgccctggcacgggtattggcaggactctccaggcgtttttaccttctctactcccagctcacacggtgccctggcacgggtattggcaggactctccaggtgtttttctctactcccatctcacacggtgccctggcacgggtattggcaggagatggagggtggctcttatccaagacattttcccatctgatcatatcccatccgcggtagccaggctccaagatggcccccatggtctctgcctcctggtgttcacacccttgtgtagtcccctcccgtatttaccagagttggtctaggtgctcctgtggtgtgggctgggtgtgagcagaagggccctttctcctctctgtctgtgtgctaggaggccatgtgcttcaatgcaa

SEQ ID NO: 15757 - RNA, 7080 nt, Homo sapiens
  source 1..7080: mol_type = other RNA
gctgggattacaggcatgagccactgtgcctggccaggatcatgtttctttaaaccacacatgatacccagaaggcatcataatagagttggcttcatcatcttccttatcctaggttatgcttgatttcaaaagaaatttgttcctcgacaatacacagaaaatgcacttaacaatagcccctgaagttttccccagccaatgactggttagcagtctaataaggatcatattggacaagtatctttaacacaaaacagcacagggaatcatgggccactctcatcgttaggctctcttcacaggtatagcctatgttagaaggcttctgaaccacagatgctaaagaaaaattagttaaactgaagactgatgaagtattccctacaaatgaaaaggcaatcttatatgacaaaggacactatcaggaggttgaaaaacaacctatagaatgggagaaaatatttgtaaatcatatgtctatgattaatatccagaatatataaagaactcctgtaagtcaacaaccatcaccacacccagttcacaaatgggcagaggaatcttatggacatttctccagcggagatatatgcacagccaaggagcacgtgaaaagatactcagcatcattagttgctagagaaatgcaaagcaaaccccaagaaggtaccacttcctagccagcaggatgtagctattaaaacaacaacagaaaatcagtgttggcaagggtgtggaggaattgcagtccgtgtgcgttgctggtgggaatgtaaaatggcatagtcattgtggaaaggagtgtggcagttcctccaagagtcgcatatagaattgtcacatggtccagcaattccattcctaggttacccaaaagaatggaaagcaggggagctggaggccattatgctaagtgaagtaactcaggaagggaaagccacattcctatgttctcaggtataagtgggagctaagctgagggtccacaaaggcagagtggaggaatggacattggagactccgaaggggaaaggagatggaggattaaaacgctacattttgggtacaacatatactacttcggtgacaggtgcaccacaatctcagacctcaccactatacagttcatccacgtaaccaaaaaccacttggacccctaaagctattaaataaaataaataaatataaacattcagtaacattatctttagaagaacactttttaataaacctgggcatgaagaaaaaaggctgaataatattccatcgtatgcgtgtgtatatccatatatatatatatatatatatatatatatatatatgcacacacacacacaatgtatatgtctagtgttaccaacttagtttcctttccttcaatattaaacgtctcatatttcccccagactttttgagagatagttgagaaataaagctgtgtaagtttagagtgtagtatgtgatgatttgatatatattgtgaaattattaacacaagttaggtgacacacctgtcacctgtcctagttatcatttttttttgtattgtagtgaaataaatgtctcatttaaaaaaaaaagaattgaaagcaggaaatgaaacagatacttgtataccaatgctcatagtagcattaagcataatagccaagaggtaggaacaacccaattgttcatccacaaatgaggagagaaaatgtggtatgtaaatataatggaatatacgtttcatggaaaagaatgtatctttcaatttttaatttttgtgggtacatagtaggtgaatatatctatgggatccatgagatgttgggatacagacatgcaatgtgaaataagcacgtcatggagaatggggtatccatcccctcaagcatttatcctttgagttacaaacaattcaattacactcttttaggtacttaaaaacgtacaattaagttgttatagtcaccctgttgtactttcaaatactagatcttattctttcaaaaattggttgaacctattaaccatccccacatcccccatactctcccaatacctttcccagcctctggtaaccatccttctactctctatgcccatgagttcaattgctttgatttttaggtctcacaaacaagtgagaacatgtgatgtttgtctttctgttcctggcttatttcacaaaatgatctccatttccatccatgatgttgcaaacaacaggatctcattcttttccatggctgaatagtactccattgtgtatatataccacattttctttatccattcacctgttgatggacatttaggttgcttccaaatctaatggaatatattattcactcataaaaagtgtgaaattctgatacatgctgttaatataacacggatgtaccttgcaagcatgttgagtaacataagccacaccccaaaggacaaatattgtatgattccacttatacaaggtacctggcacaggcaaattcatagagacacaaagtagaatggtggttaccgggggccgggggagtagggagtggggagttgttacttaatgggtagagtttgtttgtttgggaaggttctggagataaaggatgtgatggttgcacaacaatgtgaacgggcgcaatgccactaaactgtgcgcttagttgcaaggttacaataggacattttatgtatatttcaccacaataaaaataggaaaaggcaggtgatttctaaggacacaagtcccttggggttgctagttctgtcagacttttccccttgtttttctgaatgacaaggattagtagtggatgataatgagtggattcatggatttgagcaggacatgaaacaatttccatagacagagatgaaagggcatttctgacttgaaacctgggatgagcaccgatgcaggagaggcacgaaagctcacagcgtgttcagggcgtagtgaatagaggggtgcgtgccccgagcctgcagagcgggcagggatgtgtaggaaggcaccttcatcctcctcactcagcctcccagctccaggtccaaagccgccaaatcatctttcttgtcaccatcacatgataagggggagtccttccagactgccagtcaatgaagtaacacacacagccacggtcatgccagtctgagcccatcgggcgagccctgaggggaataacagtcttggtggcattgggcaagccccgaggactccatctcggggaataacagtcttggtggcatcggcgcttcaccaggcctcctggaaccatattcgggatccccaactgagtgctggaaagaccactggtcaggagcagggagcaggggtggaaggaggtggctcgtcctgaccttgacaatgagaatcctgttttaagcttcacgctgctgactaaacagaaaggccacggcacagggacagacgtgcgcatgaaatcacaggaagaaagacatttcacgaacaaatgcatcctcccaaaccagtctgaatccctccggacagggtgatgttaccacgcaactggcctggcctaatgagctggtttctgtcatccctcctggaaggttaccctgtaacacaaggcgtgcccactgacatgcagcctgatggagcaaggttacacctgtctgccttttgtgtgcacaagatcagaacacagtcaagtgaatacaaatgcaacagctgcttggggctcaaacttgcatagtctattttatttggatagagagcataaaattggctctaccaaagtctggaggctggaagtaatcataattgtaatctagtataattaccaagcctagacctttacctagtcctatttaacctccctttcacctttccaaggaatgtggagggataagagagtcactgaataagttggttggtaatactgtattgtatctctcaaatccattgtttttttttaaagaatgagatcaataaatataaattccaatattttcttccccaaagcaccatcttgtaccgctttggagaacattagagggactcacctgggtttccagagctggaaaacataagccccataatgcacccagtccccacggcgcgctgccatcttaggcccagtccccactgcacgctgtcatcttaggcccagtccccgctgggcgctgccatcttaggcccagtccccgctgcgcgctgccatcttaggcccagtccccgctgcgcgctgccatattaggcccagtccccgctgcgcgctgccatcttaggcccagtccccgctgcgcgctgccatcttgggcccagtccccgaggcccagtccccgctgggcgctgccatcttaggcccagtccccgctgggcgctgccatcttaggcccagtccccgctgcgcgctgccatcttaggcccagtccccgctgcgcgctgccatcttaggcccagtccccgctgcgcgctgccatcttaggcccagtccccgctgcgcgctgccatcttaggcccagtccccgctgcgcgctgccatcttagggttttgcttagggggcagatagaaaatagtaaatgaaaccctttcagatatttcctggccttatttagtaaacacgtctttttgaaagaactctgaatacacctgcagatttttcaaagcccagattctacacacttctaatgtcaaccttgaagggagatcgtagattgaattacagaaaggggtgctgtcaaaatgccacatcaaatataaacttcacatatgtttcttacctgaaacactcactcacactcatggaaaagcacaggaatgttctaaaaatgcaagtttatcacgaaggagacacaggaggttcagagacgatgaagcggcaagccgggaggaaagatctgagagaagccaccaggctggggcaggatttcattatatccagaattccacttgggctctgcagtttctttcttcctgagaattatttaaaagtcccctccactgcgcatattgaagacagagcccaagacgcatccaggtgcaacgtctctgctaagaatgtgtgccaggaatggggcctggcttcctcgtcgagtgcggctgtccgtgggtttcccacagtcttccctccctgaggccagaagcaggtcacgtgtaaaatggtctgctctctgctgacagtggcctgagtctcccatagtgtctgctgagctggatagtccctctccagggagctttgcaggggatgggtgatgagacatggacatggggacgaattcctctcatctggaatcgcagacacagcatggagatatgagcacgcggcatgggaaataggcttcctcagcccttcaggatcagggaacgtgccagagatgcaatgacatttggcagcagttgagagtatgagtgctcagcagcagcatctgcagactcgtgtggggacttctgtctggactcagggatgttaagagtagaaggcccaatgtcagcttctcacgtgggctgtcagcaccgcagatgataccggaagatggactgtgatgggccagcgacccctctgactgcacgcagctgtcagccaggcctggaacaggaggggcgagggggtgggctcagcctctgttagtgggagaggtcctggttggaagtttcactgaagtatcagtgttgactttctcaggtcaaatctgggccatttcatgcggtaaatccatgtcggcaggtatcagcccaagtgttttgaacatgctgcacttgtacatgcctggaccaaatgccaggctgatgagcagggaggggttgaaaagcagaagggagcccaacccaccggcgtcagcaggaggctggccctggctgtggctccccgatcagacaggcggcgtccaatggggcaccacacgactcccgccagggtggggcttcccctgtacctttcttagagctgatggtcccctgaccccactcgcagcctggaaggaggggatccctggcagagaccgggcttggcagaaaactgggcatctgcttgagaggtggaaatgctggagcatgcagaaaatctaagaacccttatttatatggggccccagaccaggaccctcgggtcagtctttctttgcccagggatggcatagcagtaacatcgcttcctgtgccctttccagtaatgtgagggcaccatctccgcccctgaactcccttcaggccacttcactccatttcctcagcctgaccacattacccctgccccagtacttggcttccctcaccatcacctaagtgaagctcacatgcacctctggagggagacaggcgcggggagagggagcctcagctggaggtgcaggaactgagtatcaatccattcacgggattgaggttctggtacccaaattcagaattttacgaaaatccaagacacttgttcattcgtgtgcaggaaaaaggtattcctagcccccaaaccacacctaacctgacagtgggcactcacttcaccttgagagggatcgatgtggtgaggaagttcaaggttgctagatggcatggaaaggaggcaatgggaaggaagtagatacccgccaggatatttctgtgaagctgttgtagcccagtgaaatgtcactctccaggtgtttttaccttctctactcccagctcacacggtgccctggcacgggtattggcaggactctccaggtgtttttaccttctctactcccagctcacacggtgccctggcacgggtattggcaggactctccaggcgtttttaccttctctactcccagctcacacggtgccctggcacgggtattggcaggactctccaggtgtttttctctactcccatctcacacggtgccctggcacgggtattggcaggagatggagggtggctcttatccaagacattttcccatctgatcatatcccatccgcggtagccaggctccaagatggcccccatggtctctgcctcctggtgttcacacccttgtgtagtcccctcccgtatttaccagagttggtctaggtgctcctgtggtgtgggctgggtgtgagcagaagggccctttctcctctctgtctgtgtgctaggaggccatgtgcttcaatgcaa

SEQ ID NO: 15758 - RNA, 1736 nt, Homo sapiens
  source 1..1736: mol_type = other RNA
gctgggattacaggcatgagccactgtgcctggccaggtttttgagaaaagaaaagcttcttattgaaagttgactcccaaggacacaggagtcaagctcaaatctgccactctgggctggcttcaaggcagtatttttattaggaaaggcttagggggtagatactgggattagcaggtggttggtggagggaaaggggaagtctggaaagtccttgggtgtgtgtacttatttctttatgttacttcataggttgcatatgcaaatttgggagaagttagtatgaaatatgtggtggaaatttgggctgtgatgtcagcaaacttgtgcacaatctccagttggtcatcctggttccaattaattttagcccactgccaactttttaaaaaacttgtgagttaaaaaaaaaaaaatactcagaagaggagggaatttcagcatctcagcaagttgtttttttttcttatctgttatcctgcaaactcagtaatttctgtcattggtttcattaactctttagggtatagtttcatcatcataattccctgggctcagggattggctgggctcagctgggtggttcttctgttccgtgtgttgttggctggagctgcagtcatctggggcttgactgggctggaacatccaagatggtgcatgctcatggatggcagttggcactagttgttgagtgggtgttcagttggggattatctgcttaggtgcccacatgttgccttttatgtgacatgagcttctcacaacacacatcccaaggaggaggaaatggaggctgctagttctggaacagtatcccttctgctagtgatgatctcagtgatgggtcaatcagggaagccaaattacctgacataggtaaggcagcctgcggtttcagggacatctggcagccaatacgtccagctgttggaagggaccatgaagacaggcttggatagatgcccagggaaagttgttggccctttgtggctattgcctttgtgagtttgtcatgaagcatctggtggtgaacttaaggtcggctgttggtcattgagggactactgaaactccttttaacttcggatcatggtctttattcagccgagtccttcggattcttgggtgatgccagttctgcagtgacctgttgtcccaggcagcagtgcattggcctgtgcctaggtaaggctggtggatggcttcatagcctaggagtaggttggacccaaggcagaaggtgagaagtagggagaagtgagatgacttaggaagggctagagacaaggcctggggtctgaaggagcaccctgctctctagggctctggaaagggcagattggaatgctgatgccatcctgcctccagcttgctctgtgacatcaggcagctactggcctgacctccgtggctctctgtaacaggaacactgcaacaatacctgcatcttccttagatggtggcattgaggacgcagtgaggtgatgcagataaaagcttgcagctcagccctgctgcattctctgtgctcaacaaatgtcaattgctacttttgttgatgacgctgggtctgtagctttatctgtagccattagcaaagaagaggggggaatttctctgttgaaataaattgccttgtagctctggtttcctcccctaaaacatgtggatgcggacacggtacaagatttgttttgttttgttttgtttttgagatggagttttgctcttg

SEQ ID NO: 15759 - RNA, 1726 nt, Homo sapiens
  source 1..1726: mol_type = other RNA
gctgggattacaggcatgagccactgtgcctggccaggtttttgagaaaagaaaagcttcttattgaaagttgactcccaaggacacaggagtcaagctcaaatctgccactctgggctggcttcaaggcagtatttttattaggaaaggcttagggggtagatactgggattagcaggtggttggtggagggaaaggggaagtctggaaagtccttgggtgtgtgtacttatttctttatgttacttcataggttgcatatgcaaatttgggagaagttagtatgaaatatgtggtggaaatttgggctgtgatgtcagcaaacttgtgcacaatctccagttggtcatcctggttccaattaattttagcccactgccaactttttaaaaaacttgtgagttaaaaaaaaaaaaatactcagaagaggagggaatttcagcatctcagcaagttgtttttttttcttatctgttatcctgcaaactcagtaatttctgtcattggtttcattaactctttagggtatagtttcatcatcataattccctgggctcagggattggctgggctcagctgggtggttcttctgttccgtgtgttgttggctggagctgcagtcatctggggcttgactgggctggaacatccaagatggtgcatgctcatggatggcagttggcactagttgttgagtgggtgttcagttggggattatctgcttaggtgcccacatgttgccttttatgtgacatgagcttctcacaacacacatcccaaggaggaggaaatggaggctgctagttctggaacagtatcccttctgctagtgatgatctcagtgatgggtcaatcagggaagccaaattacctgacataggtaaggcagcctgcggtttcagggacatctggcagccaatacgtccagctgttggaagggaccatgaagacaggcttggatagatgcccagggaaagttgttggccctttgtggctattgcctttgtgagtttgtcatgaagcatctggtggtgaacttaaggtcggctgttggtcattgagggactactgaaactccttttaacttcggatcatggtctttattcagccgagtccttcggattcttgggtgatgccagttctgttgtcccaggcagcagtgcattggcctgtgcctaggtaaggctggtggatggcttcatagcctaggagtaggttggacccaaggcagaaggtgagaagtagggagaagtgagatgacttaggaagggctagagacaaggcctggggtctgaaggagcaccctgctctctagggctctggaaagggcagattggaatgctgatgccatcctgcctccagcttgctctgtgacatcaggcagctactggcctgacctccgtggctctctgtaacaggaacactgcaacaatacctgcatcttccttagatggtggcattgaggacgcagtgaggtgatgcagataaaagcttgcagctcagccctgctgcattctctgtgctcaacaaatgtcaattgctacttttgttgatgacgctgggtctgtagctttatctgtagccattagcaaagaagaggggggaatttctctgttgaaataaattgccttgtagctctggtttcctcccctaaaacatgtggatgcggacacggtacaagatttgttttgttttgttttgtttttgagatggagttttgctcttg

SEQ ID NO: 15760 - RNA, 1663 nt, Homo sapiens
  source 1..1663: mol_type = other RNA
gctgggattacaggcatgagccactgtgcctggccaggtttttgagaaaagaaaagcttcttattgaaagttgactcccaaggacacaggagtcaagctcaaatctgccactctgggctggcttcaaggcagtatttttattaggaaaggcttagggggtagatactgggattagcaggtggttggtggagggaaaggggaagtctggaaagtccttgggtgtgtgtacttatttctttatgttacttcataggttgcatatgcaaatttgggagaagttagtatgaaatatgtggtggaaatttgggctgtgatgtcagcaaacttgtgcacaatctccagttggtcatcctggttccaattaattttagcccactgccaactttttaaaaaacttgtgagttaaaaaaaaaaaaatactcagaagaggagggaatttcagcatctcagcaagttgtttttttttcttatctgttatcctgcaaactcagtaatttctgtcattggtttcattaactctttagggtatagtttcatcatcataattccctgggctcagggattggctgggctcagctgggtggttcttctgttccgtgtgttgttggctggagctgcagtcatctggggcttgactgggctggaacatccaagatggtgcatgctcatggatggcagttggcactagttgttgagtgggtgttcagttggggattatctgcttaggtgcccacatgttgccttttatgtgacatgagcttctcacaacacacatcccaaggaggaggaaatggaggctgctagttctggaacagtatcccttctgctagtgatgatctcagtgatgggtcaatcagggaagccaaattacctgacataggtaaggcagcctgcggtttcagggacatctggcagccaatacgtccagctgttggaagggaccatgaagacaggcttggatagatgcccagggaaagttgttggccctttgtggctattgcctttgtgagtttgtcatgaagcatctggtggtgaacttaaggtcggctgttggtcattgagggactactgcagtgacctgttgtcccaggcagcagtgcattggcctgtgcctaggtaaggctggtggatggcttcatagcctaggagtaggttggacccaaggcagaaggtgagaagtagggagaagtgagatgacttaggaagggctagagacaaggcctggggtctgaaggagcaccctgctctctagggctctggaaagggcagattggaatgctgatgccatcctgcctccagcttgctctgtgacatcaggcagctactggcctgacctccgtggctctctgtaacaggaacactgcaacaatacctgcatcttccttagatggtggcattgaggacgcagtgaggtgatgcagataaaagcttgcagctcagccctgctgcattctctgtgctcaacaaatgtcaattgctacttttgttgatgacgctgggtctgtagctttatctgtagccattagcaaagaagaggggggaatttctctgttgaaataaattgccttgtagctctggtttcctcccctaaaacatgtggatgcggacacggtacaagatttgttttgttttgttttgtttttgagatggagttttgctcttg

SEQ ID NO: 15761 - RNA, 1787 nt, Homo sapiens
  source 1..1787: mol_type = other RNA
gctgggattacaggcatgagccactgtgcctggccaggtttttgagaaaagaaaagcttcttattgaaagttgactcccaaggacacaggagtcaagctcaaatctgccactctgggctggcttcaaggcagtatttttattaggaaaggcttagggggtagatactgggattagcaggtggttggtggagggaaaggggaagtctggaaagtccttgggtgtgtgtacttatttctttatgttacttcataggttgcatatgcaaatttgggagaagttagtatgaaatatgtggtggaaatttgggctgtgatgtcagcaaacttgtgcacaatctccagttggtcatcctggttccaattaattttagcccactgccaactttttaaaaaacttgtgagttaaaaaaaaaaaaatactcagaagaggagggaatttcagcatctcagcaagttgtttttttttcttatctgttatcctgcaaactcagtaatttctgtcattggtttcattaactctttagggtatagtttcatcatcataattccctgggctcagggattggctgggctcagctgggtggttcttctgttccgtgtgttgttggctggagctgcagtcatctggggcttgactgggctggaacatccaagatggtgcatgctcatggatggcagttggcactagttgttgagtgggtgttcagttggggattatctgcttaggtgcccacatgttgccttttatgtgacatgagcttctcacaacacacatcccaaggaggaggaaatggaggctgctagttctggaacagtatcccttctgctagtgatgatctcagtgatgggtcaatcagggaagccaaattacctgacataggtaaggcagcctgcggtttcagggacatctggcagccaatacgtccagctgttggaagggaccatgaagacaggcttggatagatgcccagggaaagttgttggccctttgtggctattgcctttgtgagtttgtcatgaagcatctggtggtgaacttaaggtcggctgttggtcattgagggactacttccttccgcattcatgtcatgatgctcttgcgttggtctccctgccacactgaaactccttttaacttcggatcatggtctttattcagccgagtccttcggattcttgggtgatgccagttctgcagtgacctgttgtcccaggcagcagtgcattggcctgtgcctaggtaaggctggtggatggcttcatagcctaggagtaggttggacccaaggcagaaggtgagaagtagggagaagtgagatgacttaggaagggctagagacaaggcctggggtctgaaggagcaccctgctctctagggctctggaaagggcagattggaatgctgatgccatcctgcctccagcttgctctgtgacatcaggcagctactggcctgacctccgtggctctctgtaacaggaacactgcaacaatacctgcatcttccttagatggtggcattgaggacgcagtgaggtgatgcagataaaagcttgcagctcagccctgctgcattctctgtgctcaacaaatgtcaattgctacttttgttgatgacgctgggtctgtagctttatctgtagccattagcaaagaagaggggggaatttctctgttgaaataaattgccttgtagctctggtttcctcccctaaaacatgtggatgcggacacggtacaagatttgttttgttttgttttgtttttgagatggagttttgctcttg

SEQ ID NO: 15762 - RNA, 2478 nt, Homo sapiens
  source 1..2478: mol_type = other RNA
gctgggattacaggcatgagccactgtgcctggccaggtttttgagaaaagaaaagcttcttattgaaagttgactcccaaggacacaggagtcaagctcaaatctgccactctgggctggcttcaaggcagtatttttattaggaaaggcttagggggtagatactgggattagcaggtggttggtggagggaaaggggaagtctggaaagtccttgggtgtgtgtacttatttctttatgttacttcataggttgcatatgcaaatttgggagaagttagtatgaaatatgtggtggaaatttgggctgtgatgtcagcaaacttgtgcacaatctccagttggtcatcctggttccaattaattttagcccactgccaactttttaaaaaacttgtgagttaaaaaaaaaaaaatactcagaagaggagggaatttcagcatctcagcaagttgtttttttttcttatctgttatcctgcaaactcagtaatttctgtcattggtttcattaactctttagggtatagtttcatcatcataattccctgggctcagggattggctgggctcagctgggtggttcttctgttccgtgtgttgttggctggagctgcagtcatctggggcttgactgggctggaacatccaagatggtgcatgctcatggatggcagttggcactagttgttgagtgggtgttcagttggggattatctgcttaggtgcccacatgttgccttttatgtgacatgagcttctcacaacacacatcccaaggaggaggaaatggaggctgctagttctggaacagtatcccttctgctagtgatgatctcagtgatgggtcaatcagggaagccaaattacctgacataggtaaggcagcctgcggtttcagggacatctggcagccaatacgtccagctgttggaagggaccatgaagacaggcttggatagatgcccagggaaagttgttggccctttgtggctattgcctttgtgagtttgtcatgaagcatctggtggtgaacttaaggtcggctgttggtcattgagggactatttcatctgtactgtgatactttcttctctgctgctgatgcctggtggggcaggatgctctgacctcccaggtttcaatggttttctcactgattcaccgtccctttgcatctgttcaaaaggaaaaactttctgggctgcatctttctaaagtaaaccttcccatggcttaggcaactcctgaccactgcggggaggatttccttgattgcacctgtgtcgatcttcggccatagtcattgggcagttatcttgtagttgctttgatatctaaatctcccatattagactggaaattcctagatagcaagagccatcttttaataaacaaaataataacgataaaatattaaaaacatactgagtgtcaggcggtgttctgagctgattttgagggttatttcacttaatcgtcagatatccccatgagacagggacttttgtattccccagttttcagataagagaatgaaggcacagaggggtgaaccatggtacccaaccaaggtcacatggccagtaaattgcggggtaccagcacttgagctcgggctgattccagaccgtacactctaaacgcagcactttgttcatttcctacaaactacttagcatggttgcaaaagtatcattgaatgaattaacgaacaaatgaactgtcataatctaatcacagaaattatgtccttggaggggaaggttgaagcctttataatttgccctaggggagagaagtgaagccaaagcactttctgtctgtgtatcaggaatgagatcgtgtgggagggatagtgatcagataatgagagattttctctctaaaacaggggttgaccaagtatagcccacgggccaaagtcagccctccacctgcttttgtaaataaagttttattggaacactgccatacctatttgtttccactttgtctatggctgttttcacgctgcaacatcagaattgtgtagtgtgacagagaccgtatggcccacaaaacctgaaatatttactgtcaagctttttagagaaaatgtttgctaaccctttttgtaaaagaccaagctagaaatagtgagtgtcaattaaaacaaatacatacatgtctaagtcaggggagattttggtctgatgtaaagaagaacttccttttggaggagggcaataaatacatgaagaggctggggaggcattgactgtggagaactctgtagtgggggtgaatgaatatttgcacaagtggtacaacatttatagggggctgtaattgatcaagaacttcctatagtaagtgctcaggggaaggcaggaaggaggcacacgcccagagagggtgagatgcctagggtcacacagctagtacctggtagagcttgtgctcaaacccacatcagtttcacccaaaactttcat

SEQ ID NO: 15763 - RNA, 1547 nt, Homo sapiens
  source 1..1547: mol_type = other RNA
gctgggattacaggcatgagccactgtgcctggcccaaactttttttttttaacgtagactttcagctgcatgacctggtcccagccctgtagctcggaagccccaggaggtgaggttcacacccttagggctgggactctctgagccctaaggatgagattctaagttcagagatgagttgagggcttccctgaagggaccaaggaagtccctgtggcagaaacaacaggagacaagaggtcagtggtgcggaggggaggggatggtacagaggggcctggggctggatcggagggttttggttgggaggagaagagaggggagggcaagaattcttctccaggatgggcattcccccatgctcacttgtgggtttcccctcagtacagtagggcccccccgcaaagcagcagctgcagtaggtagataagatggaagaagcttcttctggtagtttctagaacctgaagacagggcccgtcagggcctttgattggacccaggaattctcagtatgccagggaggtacaagtgcttggttggttaatgaggggtcccagccaatggtcccaggccctggaaggcacagtcaggctgtcttgcaagaagggtagtgctggactaggacagacggactcgcacgatcacactggagttggtcacacgggctccatagtggccagcccagaactgtgtgtcctggccccggtgttcgaaagacacaaagcggacgcccatcttgatgttggagaacacgtgggtgacgtgaaggcaggcattgttgttccactgcgggatgggatcaggcacagcagagaatttatctagaacagtctggttggcgtctagaagttggacgaggagtctgtacatacagccgctgtcgtgtcgggctccccaccagtcagagacacaaatctcaatcctgccactatccagcagttctggccacagaccctcctcctctaggtccaagacctgcttcttgcaacaccagctgaatgaagtcacgaagcacgtctgagaaggggccccaggcacggttgtcctgttttcctccaccacccagccgtccccaccgtgttgcaccatccactttcggaggccttcttggccgcaggggttgcgaataaggttgcgtccgatgggtctgcgcgcgcagaagcggcccagggggcaaggcctggcgttacgggcgggagactggcagctgcgggcgaggtgcagcagcgcgcggccggtggcgccgtggtcgcgggccaggatcagcagccacagggcctggccgtccaccagggctcgccagccccggcacacttggcggcagcgcccgagcagcgtgcgcggggggacgtggctcagcaccaccagaagcagctctgggggtagttggctcaggtccagcgcctcttcgggttccggctccggcgcggggacccgggcggcccggcccctggagaccgaggcgcccatggtccccccgccaggcccggctgtggcccggggcctggcggcgctcctcgccgggatgccctagctgtgccgc

SEQ ID NO: 15764 - RNA, 1340 nt, Homo sapiens
  source 1..1340: mol_type = other RNA
gctgggattacaggcatgagccactgtgcctggcccagaaggagctttgaaagttactgtgtgacatggggggctaggaggggaggcctagaatagttgcctgagactcgtcttccccgatgatgataccgcaggtgagcagggcatagaaggaggtggtctgcttgagcagcaggtaggagagcagcacgttgaagacggtggtgagtgagcggcccacattgtagaaggccacaccgacgtacttgaggcagaggttattgaaggtgatcatgccgatgaagaccaccgacaggggcaggacgctgcgggccaccctgaggtccaggcgcaagctggggaagtccacggcaccagggcagcaggcggccagagcgctgaggcctttgcacagcagcgtggtcaccaggcactggtagaaggtgacgaagatgggggtgtccagccgcagggaggggctgtccagcaggtacttattaaggaacaccatggagatggaggtgacccagtagagggagaccaccagcgcgatctgcaatgcccgcagcagaaagggcttctccccgttggcctctgcctctgcagaggggtctgaggccccggtcagcgccatgtgcaggatcctggaccgcttcagaggggccctattcatggtagcagaggagctgggtcaccccgcggccagaactctgattccctggagtccagggcagtgagctcacttgtgctctccgcaaggaagccgcagccctccattgtcacatgtgggctggcctaaaggcctccccattgtcctcatggattgagaagttctgctttggggtgagcccagttgtgctgctccacaacctactcccaccccgagggggctctgagacaagacacagggcaagggagaggaataggataaggcggtgaggccaggacagagaagacctgtgaggggagaagaggctggggcctaacagggaggggtcgcagagagaagggaggggagaggaatggcagggcggggcaggagtaggtacgcggggcgaaggtgcaggaaaaggacgcgtggcagagtgggaagaggtgccgagagggcgtcatgggcggctgtgggagggaggggcgggcagggggagggaggcgtacagggagctgccggaggccgggcgcggctggagggagggctgcggaagggtcagaggggctcggggcttggggctgaaggacgcgggagggggctgggccggcgcccacgtctcgctgccttcccgggctctgtcgccggctcagcccaggagcctccggacatccgaggccgactccccgggaggcgggccctggactcactt

SEQ ID NO: 15765 - RNA, 5092 nt, Homo sapiens
  source 1..5092: mol_type = other RNA
gctgggattacaggcatgagccactgtgcctggccccagtcaaagtttctttacaaaaacaggtgatgggtcagatttggcccgtgggcccagagtttgccaaactctgcattagcccaaaacaggggccttcacactgggtttctcaaaacttgggattgtttggaagtgcttctgggggttcacaaacgtttggctctaatttaaattatttgtaggtgtttaggaagctataataaaagcatgcactcaaatgtattccagcatttcaccatgcaggaaatcaacatattaactgtcaggtaagtaaactcctttagtgaagacctcagaatggagcttctctggctatctccatgcatatgtatgagcagtatgacaaaatggttgaaaacctgggtcctagaatcagatggacatgagtttgagtcccagcactgccacttactagctctatggctttggacaagttactttgcctccctaaaccagcatggccaggacaccacaaaacagagtagacactggccatagtgccgctgcagcctcctagaggctgcattgtgggaaaatggagcgctcacagtggaaaggtcagctgaggccacgaggagacattcaggggactcagcgcagcattatctaccaactgctatggaggtatttcaagttttagtcatcagtttggctgtactggtgcacaccaattgagtgtcattataatgccaaatccatcttggctttgaacttcttgctagtttctatttttttctggcacattctgatatatccccactactctgattgggctctcagataggagagggggatgttttgcaactggctgagcagtctcagtgcttagtaacagggcttccatttttctgctaagcagcagtcccattggctctgggattttgctggcaggcatctcctggaaccagtgttctgcagggcttgttggggaagtggtgctctcagctaaaggggtccagtgtttcagaagccgtggctgctccacctcagtgctgcattccctggttaggcctgggactttggtgttcacctggctttttaatttactggtgaacaacactcaatgttcctcatccctgggcacctcctcacctctaagacaatcagaaggcccgtgtaactgctgcctaagactgcccctcagatttctggctttttattccagtgactgaaagcttttttccaggcctgagatgctcatttgtgatttcaataatagaatttagactcttagtgtttctccattgcccagggctgtctgtgtctattaatgatggctccagtgaaatccatggcttttactgcaccttatctttctgcttccagcatcatattttcctgcttcctgagagacatggaatcatcagtggtgttcatcaccaggccctgggggcaagaccacacaggtcccagaatccctgcagtttttcttaattaggtgacatctggtgccgtccccagtgcacaggtccaccctggtcagtcagcctgttgccatgctgtgagcctgggctgtgcccggccttgtaggcttcttgcagtcactggttctgtgagccttggaggctcttccacgggggtgattctgacccctgggagtgagaaggagagggcctttctgcagttcagccaagaataaaggagactcagggctgagctccctccttcacttcttttttgtttccttgaggttgttcttggccctcacagtacctctgtctaggcttggagctctggaagtagacacaacccgggtcttctgccccaaggcctcctctgttagccagaaggatcctggctgtgcagtggaaatgacctcgtgcaaagacattatcatatgcccttccaggggcaataatgccagtgtcccctgataaagcagtcactgtgggtatctgtcccagtcactccacacagccatacccttcctccctgggaccagcctcatggagacctctgacaatgacagtaaaaactcagcccagcctttctcttctggcccaaatcgttgctcatttgagaaccgtctctgccttctcactttgttctccttcctggaatatctttctgcatctcttaccctgccccacactgcacagaacctgtgccctttcagaccctgagctgagtccccagaaggacaaagatcaaaaaccccagggtgttctcttcccctatttcctaccaccacatctccaggcttctgcccctctcatgatacttttggttttctttacaaagtgcttgctcatgactaggattcctcctagaagcctggcaatcagtccacacacagatgtctgctcaccccttctgtctccctggggaccagccattggtgcttccaccctccctctggagagagccagggatgctcagcaaaggaggaggctgactcatcaagcggtgagagttctcctctgaaagtggtgaagaaggggccgcaggggctcttgcaaatgtggaggatccgctgatgcatttcatggggaggttatctcatcctggaagcccttgctcagcatccactgatggagagctcattacctccaaaggcagctctgactggctttccactaacaatcccatagctggagaattttgctagtgcacatttcagctccttcctctccaagcatcactgtctcagtaccttctgtctcacaccagacctcctgacacttcccacttcaccccaggcagcacctcaccctggggctcagcctggacaaccgcctacctcagccactgcactttcttcccctagaattgaggccacaacagtagacacccatgctctgtcccgttccccaccagcagagctgctcaacaggatgcaataactggaggaatgagggtggtggaagtgagggtcttggcaggcaagagcaactgaacttcggctcaaagcaagagcaaaggaaacactgagcaggcagctactaatgcttctcccgggaagagcctgcagtgccccctgctggctggaggagagtttgtatgcgtgtccaattcactccccttgcttcctgggctgagccctgatgaccattcaggttagagaatcacatgagcagataggtcatcttgtccagtggtttcaaaatgtgtaaaattatagatagagttgctgggggcgattttgcattttgtccatttgagaaaggcctctgagctgaggggacacatgggggctgaaatccagcctctatcctgctaactaagctgtgtaccccactatgggactgggtcaggccagaggaagggatgtctttttgttcttcattcacctagacagtgtccttttgtaatttgcacaaaggtgccatacataccagcagcagcactgacacagaatgcttccttctaagagggcgatcttaaagaaccaagcttctttggctaaaagggagcttgaaaactgcccaaaagatggggaaactgggggccatgaaggggagggattactcaaagtcatgcagttaataccaggacagagcttagaagccagatccactctctcccatagcagtgttgtttacaccacattgagctagttttcatcctaagtcactattgagaaatcctggcttctctgaccctccccctctcagacccattaacttcccccctgaaatccagctactctgcacagtcctactctcctactcaggatcatggcacagaatttgccccaaaggagggatgttgagaatgccagacccgtctgcataatttcctacaagtacatcactcatagggatgagggcagacaggcagaaggacagaacagtgagaaactagagggatctaccagaggaggtgtcgaagtatgtcagggagcctggagcaatgtggatcagtaaagccggtggttcagctactgtgcagatggggcctgctttgcaggtgcagtccgccggggtgtctgtgccacaccataaggcacatgggcggccacagtgcccatctcctgagccccagccacatggaacatctggtcatcaaagaagatgtgtgggcggatcttctcaaggagagggcccttgggcgctccagcaaggaacaaggcttcatctgtctccaggccccagctgcgcagggtcttgagagcccgggccccggaactggctgcactgcgtgctgtcaccaagtaggtacgaattgggcactccagccgcaggcctttggagtagaacttcttctgcaacctacccagtgcctccagaaagccctttaaggggccctgagccagaggtttgttctcgtgggccttctcatgctcgaagaatcggtccagcccgtgggccttgacgatgcgctccgactcgtccgagaagagcacggcgtccccatcgaaggccacgcgcagctgactctgggacacaaccacatccctgctggggctgaagatggtggcagctgcgatcccctcatcaatggcttctcgcactttttccgcatcggctgacaagtagaggttggtgtgataggccttgaggtagcagatcgggctgttcccacctgtcatgcagaacctctcgatgaacaggtcatagtggttgatactgttgatgaggcggacacccacttgagcatggttgttagtcatgaggacgatgtcgaagacgtcctcactatcagggtacagctcccgcagccgcctgttcacggcctccagagccttcacaaaagggaaggctggcccgggactgaagggttcgttctcatgttccagctggtagcgcacgtactcctccacgccctgctccgtgtagatctgctgctcctcgtccatgcgaaacaaggctcgggaggacacagcgatggtgactgcattctgaggcttgggcgatttgggtttcttcttgggcgcgaggttgtcgtagaaaatcttggcttcctcccagaccggggccgcagcggtctccgctcctggcccgggctcgcggggctcctggggctcccggggctgcccaggttccatgctccggctctgacccggcccggccagagcaggcggcggcgtagacgcggaggtggctggggctgggct

SEQ ID NO: 15766 - RNA, 1146 nt, Homo sapiens
  source 1..1146: mol_type = other RNA
gctgggattacaggcatgagccactgtgcctggcccccatttggatcctttaaaacatcctttgtgataaattgatcaacataagtaagtgtttccttgtgttctgtgaacttctctagcaaattaatcaaactcaaacagaggactgtggaaacctcaactcgaagccagtcagtgagaagttctggaggtgtggagtttcaactggttggaaggaggaggtgttcttgtgggactgagctctcaacctgtggttgctgaggccatttccaggtagacagtgtcagaattgaattgaattggaggacttccagttggtgtctgctgcagaatagattgcttgcttggtgtatggagagaaacgtgcacacatttggtcacagaagtcttccgtgttgattgttgtccttgtgctgccagtgtacaaagatggggtcagctctcgctccttcaagttcttccaaatagtctatgcttggcttccttttggaggtttccagatattcttttaacggatacatgacttaatatgtcatcagcacaacattttcacagactgctgggcagaatttagacagcttgaggaagtgatgacaatggctgggggctccattcctccctgtttctgctcatcacagctgcacatctgggctgtcagcccctgagcagccaacaagatcaggagtggggtgaacacagcacatggccaaggcagtggagacttgtttactgtcgccatgggaacctctgaaggtgctttaagggggtggagccaaaagctggggcagagtcagaacagctggggcagccacacgtctctgacccctcccaacctagcgattttgggaagcctttctgcttggctctttagacccagcttgcccctctgtcctggaaatgagcctcaattattttctctccaaaatttgggacatgtggctcccctgggcagatggtggtgagatgggtgagaaggaaccaagggcggagggagacaagggctgttgcagggtgggtctccctggatcaggggccactggagaagaacttcctgtgatggaacttcacaaatgggggtggggaagcatgaggtcacaagggtcagattgtgaccacctggagtgaagctcaggatttgccagccag

SEQ ID NO: 15767 - RNA, 1073 nt, Homo sapiens
  source 1..1073: mol_type = other RNA
gctgggattacaggcatgagccactgtgcctggcccccatttggatcctttaaaacatcctttgtgataaattgatcaacataagtaagtgtttccttgtgttctgtgaacttctctagcaaattaatcaaactcaaacagaggactgtggaaacctcaactcgaagccagtcagtgagaagttctggaggtgtggagtttcaactggttggaaggaggaggtgttcttgtgggactgagctctcaacctgtggttgctgaggccatttccaggtagacagtgtcagaattgaattgaattggaggacttccagttggtgtctgctgcagaatagattgcttgcttggtgtatggagagaaacgtgcacacatttggtcacagaagtcttccgtgttgattgttgtccttgtgctgccagtgtacaaagatggggtcagctctcgctccttcaagttcttccaaatagtctatgcttggcttccttttggaggtttccagatattcttttaacggatacatgacttactgggggctccattcctccctgtttctgctcatcacagctgcacatctgggctgtcagcccctgagcagccaacaagatcaggagtggggtgaacacagcacatggccaaggcagtggagacttgtttactgtcgccatgggaacctctgaaggtgctttaagggggtggagccaaaagctggggcagagtcagaacagctggggcagccacacgtctctgacccctcccaacctagcgattttgggaagcctttctgcttggctctttagacccagcttgcccctctgtcctggaaatgagcctcaattattttctctccaaaatttgggacatgtggctcccctgggcagatggtggtgagatgggtgagaaggaaccaagggcggagggagacaagggctgttgcagggtgggtctccctggatcaggggccactggagaagaacttcctgtgatggaacttcacaaatgggggtggggaagcatgaggtcacaagggtcagattgtgaccacctggagtgaagctcaggatttgccagccag

SEQ ID NO: 15768 - RNA, 4133 nt, Homo sapiens
  source 1..4133: mol_type = other RNA
gctgggattacaggcatgagccactgtgcctggccggctgttatacttattcttgttagctacaggggaaaaaaaacaatggtaggaggtttcagagaggaagctcagcacttacaaggaagaactgctcaacagttttttccaaaccaatgttctgcagcgtacatgttaatttaaacaaggtatcttgtgtctttactgcaggatatctcagagtctttaatatgcaaatgttaagaaaaggatacagtatgccacatttcccaaacttatttgtccatagacacttctatttacagaactgtgttaatgtctcttgaaacaatggtcatagaacagtttgggttaaagctatttaaaaatgaacaggctgtcttctaaaggagtagggtcaggttcacatcaagatatctggaaaaactggttggtctggctgccgctcttatatttctgaaatgcttgtcattaaaactgaagtatataaagtttgggcacttagagcaatttctcttacctgttaacagtaacattatctgttaatattaacaggtgcctgttaacatgaacattgttacgtattaacattaacagtatgagacccaacactgttctacatgagaataatgttttaaaaccaatggaaatgaagctctctagaacagtgattctgaacttttttcctagtaacacactgcacagtcgtgccattcccgtgtctgtcctctgattcattcattgtgtatgaggtaatgtttctcaattttttttcatgaccatacacatacacaaacaaaaccctcatgctctaccatccctactcccacaaattttgataggaacctcacataggaccatgctcctctattgacatttccattttagaacctcaaacctagagcattaatgtaactttttttgaataaaaagaaaatttctaggcttcaaggcagaaatggtatttaaaacttatgggaaaagtaaatcaggaaaacaacatcaaaaaggaactactttgatatttttgaggctaaatggaaacattaataaaggaagttggacttatagaaacattgttgttattgaatatttgctgcaataagcaagacaaggtgtaataataagaaaaagctggatcagcaaggttgacaagacaaggttgcaaattataattattgtttatacaactgttcactgaagggcatagaccagcgccatagaggctaagaagaatgtactctgtaaaagaatgactggctcttcaggatttctacaacttacacctgttcctgttctccagaacaatgtttactaatgcttactatctctaatctggtttccatgatctatccatactgagaaaggagggtttggataagtaaataaaatactatcataatcagagagatataacttctcctgtgttttaataaaatggcattctgcttcctaccatctatattgacaaatttactaaagtcatatcaaacctagagagctgacaagccaggccctggctggaccagatcacatcatacataccaattcttgaggcccctgtgaatagcataattacattgcttataaaaaaaaaaacttgaaataccatttctttgttattctgcaattttgcctctaaatcagcacctcaaaaattagggccatcagtcctaaatggcagttacctataaaggaattcccataactttgcatacccacagagaatgatctccattatacgtgtgtattttcatggtcatttggagacaccaggccagctccagcaacactgcacaagttttaatgagttcactgatggacgggcagacatagagtctctggggccttgtttaaagatgtactggaaaaccagtcctggaacttctgtcattggagaaaggtggaggagatcagctctgatatgctgctatctctcttgtctaatccagtagaagaaaaaaaatgcttcaagacagggccaggaattggggtcaggacagaatctagggagtcatcagagttttgtcttcttggtctctagtttgatcatgttcccctggatgtgaggaatgtgcttatctgctggaccccgcatatcctctgtctttacaggaacatagtagtagcccatgatggagaagatcaggcagatcaccagcaggaggcaggaaaacaaaatgaattcggcccactgagaataagaaaactcaagacctgtgacagagaacatgacctccccagctgtaaccagggcatattgtggtagctgccacgcaatggacattttgttggctggaatgtcttcaatcttccaggcctgaagaccctgattggtgttattagtaataacaaacagatatgctgcaccaaagtctagaagacccaaattcagagaaaagttcttatcttctgttctacagtgcactgcagggtattctcctctttgcacagttctataagcagacacaccatagtcttcaccaacattgagagaggtatctgtactcagggagatgttgacatctttatgcaaagtgttaacaaacctcacggttgtcatcccattggttgttctgctttctgtatcctttaccatcatgctggagatactgttcccatcttcacgaatgacaagactgtaccagttcttctcctgcacagaatgctcagtgtagagagacaaattgtgatatttcaggtggaagtgaaaatcctggctttttgttttcaggtgcagtttggaatagtgtggtgttttctgaaaggatttgatggactctatcaacagagaattgttttcatttcccaccactgtcaccttcacctcatcatctgccagattcaagacttgtaggaaaacctcctggggacctggctgggctggggccatttcatttatttttatctctacagctgccgcaactgcaaatgccaggcatgctaggatcataccaacagccattttcctaagtgatgagaagttaattccacacttggagaccagacgataaatgacaaagtcaaacaacgggatgaagataagaaccagaaggggatttagaacctgcatctggtccggctgaagcacaaaaaaccccaaattcctattcatcctgatggcttgcaaagtccatcgtgaaccctgctgatccaaaagagcccagaacatgggcaatgggatataaaggaatagtaccctggtcagtgcctttacatccataatgagctgctttggatatttctcagccgcccagtctagccagtgctgtcgctttggaatgtctccagaacggttcttgaaacgattggaaatagcaaaccagatacatttgaaaacttgagccactatgtttccttcagggggtggtttattgtatattttgcttcccattgcaaacacaacaagtgcaattaccatgagcagtcctggaactccaaaagccaatgcatagcagtcttctccaaaacattgcacatctcctctcagcatgggtgtgataaatgtagaaatcaagctccctgcattgatggacaggtagaagactgagaagtatctagtccgttcctctgcatgtttttcttcaaactggtctccaccaaaagctgccacacagggtttgatgcctcctgtccccaaagctattagactcaggccgatcaatgataggactgtgtgtaccacttgtcctcccagtattggtaaggcacccaaggacttgatcacatggccaagcacatacaccaaggagagatagatgattgtcttgaattttcccaaccacgagtcagcaatggctgctcccaggatgggagtaaaataacagaggctgctgaaggcatggtatatagatgtggaggtatcttcattccagtgcaggaaatacaggaaatacaggatcagcacagctttcattccataataggaaaagcgctcgcagaattcattcaccacaatgaaggcaatgctcagtggatagttggagccacagattgtcggagatggcttctttggagggctaggtggtcgaggtggtacctcttcaatggagacaggtgaaaaaagagtttccttggactcatttttctggaaaggattcatggctggctccttactctctctctctcctcaagcattt

SEQ ID NO: 15769 - RNA, 4277 nt, Homo sapiens
  source 1..4277: mol_type = other RNA
gctgggattacaggcatgagccactgtgcctggccggctgttatacttattcttgttagctacaggggaaaaaaaacaatggtaggaggtttcagagaggaagctcagcacttacaaggaagaactgctcaacagttttttccaaaccaatgttctgcagcgtacatgttaatttaaacaaggtatcttgtgtctttactgcaggatatctcagagtctttaatatgcaaatgttaagaaaaggatacagtatgccacatttcccaaacttatttgtccatagacacttctatttacagaactgtgttaatgtctcttgaaacaatggtcatagaacagtttgggttaaagctatttaaaaatgaacaggctgtcttctaaaggagtagggtcaggttcacatcaagatatctggaaaaactggttggtctggctgccgctcttatatttctgaaatgcttgtcattaaaactgaagtatataaagtttgggcacttagagcaatttctcttacctgttaacagtaacattatctgttaatattaacaggtgcctgttaacatgaacattgttacgtattaacattaacagtatgagacccaacactgttctacatgagaataatgttttaaaaccaatggaaatgaagctctctagaacagtgattctgaacttttttcctagtaacacactgcacagtcgtgccattcccgtgtctgtcctctgattcattcattgtgtatgaggtaatgtttctcaattttttttcatgaccatacacatacacaaacaaaaccctcatgctctaccatccctactcccacaaattttgataggaacctcacataggaccatgctcctctattgacatttccattttagaacctcaaacctagagcattaatgtaactttttttgaataaaaagaaaatttctaggcttcaaggcagaaatggtatttaaaacttatgggaaaagtaaatcaggaaaacaacatcaaaaaggaactactttgatatttttgaggctaaatggaaacattaataaaggaagttggacttatagaaacattgttgttattgaatatttgctgcaataagcaagacaaggtgtaataataagaaaaagctggatcagcaaggttgacaagacaaggttgcaaattataattattgtttatacaactgttcactgaagggcatagaccagcgccatagaggctaagaagaatgtactctgtaaaagaatgactggctcttcaggatttctacaacttacacctgttcctgttctccagaacaatgtttactaatgcttactatctctaatctggtttccatgatctatccatactgagaaaggagggtttggataagtaaataaaatactatcataatcagagagatataacttctcctgtgttttaataaaatggcattctgcttcctaccatctatattgacaaatttactaaagtcatatcaaacctagagagctgacaagccaggccctggctggaccagatcacatcatacataccaattcttgaggcccctgtgaatagcataattacattgcttataaaaaaaaaaacttgaaataccatttctttgttattctgcaattttgcctctaaatcagcacctcaaaaattagggccatcagtcctaaatggcagttacctataaaggaattcccataactttgcatacccacagagaatgatctccattatacgtgtgtattttcatggtcatttggagacaccaggccagctccagcaacactgcacaagttttaatgagttcactgatggacgggcagacatagagtctctggggccttgtttaaagatgtactggaaaaccagtcctggaacttctgtcattggagaaaggtggaggagatcagctctgatatgctgctatctctcttgtctaatccagtagaagaaaaaaaatgcttcaagacagggccaggaattggggtcaggacagaatctagggagtcatcagagttttgtcttcttggtctctagtttgatcatgttcccctggatgtgaggaatgtgcttatctgctggaccccgcatatcctctgtctttacaggaacatagtagtagcccatgatggagaagatcaggcagatcaccagcaggaggcaggaaaacaaaatgaattcggcccactgtaccaggccactgaactgtgccacaacaagcacgatgatattcccaactgcaattgtcaatagccaagctgcctggagcacagatttcatgctagagggagcctgagaataagaaaactcaagacctgtgacagagaacatgacctccccagctgtaaccagggcatattgtggtagctgccacgcaatggacattttgttggctggaatgtcttcaatcttccaggcctgaagaccctgattggtgttattagtaataacaaacagatatgctgcaccaaagtctagaagacccaaattcagagaaaagttcttatcttctgttctacagtgcactgcagggtattctcctctttgcacagttctataagcagacacaccatagtcttcaccaacattgagagaggtatctgtactcagggagatgttgacatctttatgcaaagtgttaacaaacctcacggttgtcatcccattggttgttctgctttctgtatcctttaccatcatgctggagatactgttcccatcttcacgaatgacaagactgtaccagttcttctcctgcacagaatgctcagtgtagagagacaaattgtgatatttcaggtggaagtgaaaatcctggctttttgttttcaggtgcagtttggaatagtgtggtgttttctgaaaggatttgatggactctatcaacagagaattgttttcatttcccaccactgtcaccttcacctcatcatctgccagattcaagacttgtaggaaaacctcctggggacctggctgggctggggccatttcatttatttttatctctacagctgccgcaactgcaaatgccaggcatgctaggatcataccaacagccattttcctaagtgatgagaagttaattccacacttggagaccagacgataaatgacaaagtcaaacaacgggatgaagataagaaccagaaggggatttagaacctgcatctggtccggctgaagcacaaaaaaccccaaattcctattcatcctgatggcttgcaaagtccatcgtgaaccctgctgatccaaaagagcccagaacatgggcaatgggatataaaggaatagtaccctggtcagtgcctttacatccataatgagctgctttggatatttctcagccgcccagtctagccagtgctgtcgctttggaatgtctccagaacggttcttgaaacgattggaaatagcaaaccagatacatttgaaaacttgagccactatgtttccttcagggggtggtttattgtatattttgcttcccattgcaaacacaacaagtgcaattaccatgagcagtcctggaactccaaaagccaatgcatagcagtcttctccaaaacattgcacatctcctctcagcatgggtgtgataaatgtagaaatcaagctccctgcattgatggacaggtagaagactgagaagtatctagtccgttcctctgcatgtttttcttcaaactggtctccaccaaaagctgccacacagggtttgatgcctcctgtccccaaagctattagactcaggccgatcaatgataggactgtgtgtaccacttgtcctcccagtattggtaaggcacccaaggacttgatcacatggccaagcacatacaccaaggagagatagatgattgtcttgaattttcccaaccacgagtcagcaatggctgctcccaggatgggagtaaaataacagaggctgctgaaggcatggtatatagatgtggaggtatcttcattccagtgcaggaaatacaggaaatacaggatcagcacagctttcattccataataggaaaagcgctcgcagaattcattcaccacaatgaaggcaatgctcagtggatagttggagccacagattgtcggagatggcttctttggagggctaggtggtcgaggtggtacctcttcaatggagacaggtgaaaaaagagtttccttggactcatttttctggaaaggattcatggctggctccttactctctctctctcctcaagcatttggctttagtaggcagttaggacagctgccagcctactct

SEQ ID NO: 15770 - RNA, 4184 nt, Homo sapiens
  source 1..4184: mol_type = other RNA
gctgggattacaggcatgagccactgtgcctggccggctgttatacttattcttgttagctacaggggaaaaaaaacaatggtaggaggtttcagagaggaagctcagcacttacaaggaagaactgctcaacagttttttccaaaccaatgttctgcagcgtacatgttaatttaaacaaggtatcttgtgtctttactgcaggatatctcagagtctttaatatgcaaatgttaagaaaaggatacagtatgccacatttcccaaacttatttgtccatagacacttctatttacagaactgtgttaatgtctcttgaaacaatggtcatagaacagtttgggttaaagctatttaaaaatgaacaggctgtcttctaaaggagtagggtcaggttcacatcaagatatctggaaaaactggttggtctggctgccgctcttatatttctgaaatgcttgtcattaaaactgaagtatataaagtttgggcacttagagcaatttctcttacctgttaacagtaacattatctgttaatattaacaggtgcctgttaacatgaacattgttacgtattaacattaacagtatgagacccaacactgttctacatgagaataatgttttaaaaccaatggaaatgaagctctctagaacagtgattctgaacttttttcctagtaacacactgcacagtcgtgccattcccgtgtctgtcctctgattcattcattgtgtatgaggtaatgtttctcaattttttttcatgaccatacacatacacaaacaaaaccctcatgctctaccatccctactcccacaaattttgataggaacctcacataggaccatgctcctctattgacatttccattttagaacctcaaacctagagcattaatgtaactttttttgaataaaaagaaaatttctaggcttcaaggcagaaatggtatttaaaacttatgggaaaagtaaatcaggaaaacaacatcaaaaaggaactactttgatatttttgaggctaaatggaaacattaataaaggaagttggacttatagaaacattgttgttattgaatatttgctgcaataagcaagacaaggtgtaataataagaaaaagctggatcagcaaggttgacaagacaaggttgcaaattataattattgtttatacaactgttcactgaagggcatagaccagcgccatagaggctaagaagaatgtactctgtaaaagaatgactggctcttcaggatttctacaacttacacctgttcctgttctccagaacaatgtttactaatgcttactatctctaatctggtttccatgatctatccatactgagaaaggagggtttggataagtaaataaaatactatcataatcagagagatataacttctcctgtgttttaataaaatggcattctgcttcctaccatctatattgacaaatttactaaagtcatatcaaacctagagagctgacaagccaggccctggctggaccagatcacatcatacataccaattcttgaggcccctgtgaatagcataattacattgcttataaaaaaaaaaacttgaaataccatttctttgttattctgcaattttgcctctaaatcagcacctcaaaaattagggccatcagtcctaaatggcagttacctataaaggaattcccataactttgcatacccacagagaatgatctccattatacgtgtgtattttcatggtcatttggagacaccaggccagctccagcaacactgcacaagttttaatgagttcactgatggacgggcagacatagagtctctggggccttgtttaaagatgtactggaaaaccagtcctggaacttctgtcattggagaaaggtggaggagatcagctctgatatgctgctatctctcttgtctaatccagtagaagaaaaaaaatgcttcaagacagggccaggaattggggtcaggacagaatctagggagtcatcagagttttgtcttcttggtctctagtttgatcatgttcccctggatgtgaggaatgtgcttatctgctggaccccgcatatcctctgtctttacaggaacatagtagtagcccatgatggagaagatcaggcagatcaccagcaggaggcaggaaaacaaaatgaattcggcccactgtaccaggccactgaactgtgccacaacaagcacgatgatattcccaactgcaattgtcaatagccaagctgcctggagcacagatttcatgctagagggagcctgagaataagaaaactcaagacctgtgacagagaacatgacctccccagctgtaaccagggcatattgtggtagctgccacgcaatggacattttgttggctggaatgtcttcaatcttccaggcctgaagaccctgattggtgttattagtaataacaaacagatatgctgcaccaaagtctagaagacccaaattcagagaaaagttcttatcttctgttctacagtgcactgcagggtattctcctctttgcacagttctataagcagacacaccatagtcttcaccaacattgagagaggtatctgtactcagggagatgttgacatctttatgcaaagtgttaacaaacctcacggttgtcatcccattggttgttctgctttctgtatcctttaccatcatgctggagatactgttcccatcttcacgaatgacaagactgtaccagttcttctcctgcacagaatgctcagtgtagagagacaaattgtgatatttcaggtggaagtgaaaatcctggctttttgttttcaggtgcagtttggaatagtgtggtgttttctgaaaggatttgatggactctatcaacagagaattgttttcatttcccaccactgtcaccttcacctcatcatctgccagattcaagacttgtaggaaaacctcctggggacctggctgggctggggccatttcatttatttttatctctacagctgccgcaactgcaaatgccaggcatgctaggatcataccaacagccattttcctaagtgatgagaagttaattccacacttggagaccagacgataaatgacaaagtcaaacaacgggatgaagataagaaccagaaggggatttagaacctgcatctggtccggctgaagcacaaaaaaccccaaattcctattcatcctgatggcttgcaaagtccatcgtgaaccctgctgatccaaaagagcccagaacatgggcaatgggatataaaggaatagtaccctggtcagtgcctttacatccataatgagctgctttggatatttctcagccgcccagtctagccagtgctgtcgctttggaatgtctccagaacggttcttgaaacgattggaaatagcaaaccagatacatttgaaaacttgagccactatgtttccttcagggggtggtttattgtatattttgcttcccattgcaaacacaacaagtgcaattaccatgagcagtcctggaactccaaaagccaatgcatagcagtcttctccaaaacattgcacatctcctctcagcatgggtgtgataaatgtagaaatcaagctccctgcattgatggacaggtagaagactgagaagtatctagtccgttcctctgcatgtttttcttcaaactggtctccaccaaaagctgccacacagggtttgatgcctcctgtccccaaagctattagactcaggccgatcaatgataggactttgaattttcccaaccacgagtcagcaatggctgctcccaggatgggagtaaaataacagaggctgctgaaggcatggtatatagatgtggaggtatcttcattccagtgcaggaaatacaggaaatacaggatcagcacagctttcattccataataggaaaagcgctcgcagaattcattcaccacaatgaaggcaatgctcagtggatagttggagccacagattgtcggagatggcttctttggagggctaggtggtcgaggtggtacctcttcaatggagacaggtgaaaaaagagtttccttggactcatttttctggaaaggattcatggctggctccttactctctctctctcctcaagcatttggctttagtaggcagttaggacagctgccagcctactct

SEQ ID NO: 15771 - RNA, 1886 nt, Homo sapiens
  source 1..1886: mol_type = other RNA
gctgggattacaggcatgagccactgtgcctggccggttacacttatttctatcagcaggattttgtgccatcctgttgtacagctcagcaaaatacatttctatgtgccacagtcctttagaatcacttctgaatatgtgaagtcaatgttaaaactactgctgcaaagggtctgctgtagtcagctaaccttttctgttgggtctagtaggtctggacaaaacatctccctcttttccttttatattttcctcatcctcttcttgcagcgctggttgaaaacaggggaggaccccatgaggctgtcagtggagtgggaaccatagctgctatctgagtcatcagggctctgaggaatcccagcttcactcatgcctgacataggctcctcgaagacatcactgcccagcacaccatgcccagagacattgccttcttcactttcttgaggctccattttcacatgggccagattccaaagaggagaagcatttacctctgcacttgaagcctgtggtgaagcttcaacctccaggttagatgggaagcgttcgctctgagccccaagcactcccataggcagtgactggtctccagaagcaaggtcagcctccagctcctcactgacaggaaaagtgatgtcgctcacaggttcctccttgatcttcacaggtttagcgtcctctgtggccttctcaggattgacaatcctttcatattcttcagagagttgcttactaatctgtagcatgtaactgtgatagtccttgatgcggtgctgccagaacttctggagggagagcacactgccaatacccacttcatggaatacctgctccatcacatcaggaaaaggagtctgtcccagccgggcctcccggtccacagcaaaacgcagcaacttggtaaacttaaggcaatactcatgtgccacatcagttagggtctccaggacactctcattagcacagtcaaagcccgcgtgggccaggattgtggccactgcctggtagaggagctgccgacaggagtgccagctgagttcagtcacaggttcccctttcccacgataaaagtcactctctgggtcactgtgccggatctggaatggtgcattgggattcttacaatctaaaggcaggaggtcatcagggagaggaggtgacccagggcacgagggaagaggttcactctcttcagtttttacaccttctgtctgctgctgattctgggcctgagctgtggcaataaggttgcgaagacgtcggttgtgctgaatcaactgaatcgtatggatggtgagactacatggctctgaggggatgtccagcatagtggggggcttcggcttgttggctgagggttggtgcaggggtgggtcatggacttccaccagacggaactcccgtgggagcaaatcgaaggaacttctgttggtctggcttgatgatattggtatctctccccagtatctttgcagattcattgtccatatgtctcttcaagttcaacaaacatttatcaaatgccaggcattctgtgtcggtcaaagactgataatgtgagatccttgcccgaaaggagcacgaagaacaggcacggagcccaaggaatgcccaagtccctccaggggtttcctcggtcacggtccgccggcgcaggcgccaatcacagggtcctgaggtcgcctgacgttcagggcagccggaagacggggaggtctggacctgaaccgagacaaggaggtaccacactattcactgctgcgtcgcagagcgggctgggcggctgtctggacctcgagaggcctgaggcaaggatcgcgtcagaccccgaaagctggtttgttgattagtgatctaagaccgccggaagcgcttcttct

SEQ ID NO: 15772 - RNA, 1334 nt, Homo sapiens
  source 1..1334: mol_type = other RNA
gctgggattacaggcatgagccactgtgcctggccgtgatttttaagagttggtcagatgatctggagtagcttggtccaggcaaacagaaagtgacctttgtcaaatcatgaagggttctgttttgttcagtactgaagattcctttgtactcttggctgtgacctatccctgaggtatcctgagttctggaatctataagattcctctagtttttctggctgctgatagcccaagtcagactgtggtaccagcgtgacagctcctcctggtctgtggacataagcagtagcttctcatgagggaaggacagactgagcaacccaccacaagggcctcctgagtggccaaagaccctgctgagatgacactgggccatggggtagagggccttgcaggcaaaggtgccactccgcagcaggtgcagtggaggccgaggcttggccatgaggagcacatcagtgaagaggaagaacatgcggggccgaggctccccatggggaggcaccactaacagccagccctggcgtaggaaccagcgccctgaggtcagcccctttgcctggcgtccactgagcagagcctggacacgccgaaggtgctggtcattcttctgtttctgaccaatagtatggactctctgggcagtctcacttatcagtcgggcagccccagacattgttggaggtcagaatcagaaaggaatacaggagaggaagcctccagcctgcgttgccgaggagcaagaacctacgtgtgagctgttgatggtcagggctgttgggacctgtgttttcagccaaagctacgacgagattctcatactgctggagccgttgcagaggcagagggagcaggtcctggagctgaaggcccccaaactcagggcggccttcctgaagccgtacaaacctccggaaacctttatttttctttagctgctcctgcagggtggtctgggacctctctgagttggcagcaaattggttatagagctccaagtggcggcagaagccctccagcccttggccccagcatcctccttccaggtagggaagcagctcctggctggcgccgtagatgagctcccaggagccaaacagggcctggcgctcaggtggtcgcagggtccccttggctttcaggatccccaaaaagtacgtggccaccagccccagctgttcttggtagcgccgctcggtctctagcagctcccgggcggtgcaggcgcgtttccgctcccagcgggcacgctgctcttgcaccgggcaccgcgaaccggggcaggagagctccatgccctggctgagggatcgacacttccggctgcagtc

SEQ ID NO: 15773 - RNA, 1242 nt, Homo sapiens
  source 1..1242: mol_type = other RNA
gctgggattacaggcatgagccactgtgcctggccgtgatttttaagagttggtcagatgatctggagtagcttggtccaggcaaacagaaagtgacctttgtcaaatcatgaagggttctgttttgttcagtactgaagattcctttgtactcttggctgtgacctatccctgaggtatcctgagttctggaatctataagattcctctagtttttctggctgctgatagcccaagtcagactgtggtaccagcgtgacagctcctcctggtctgtggacataagcagtagcttctcatgagggaaggacagactgagcaacccaccacaagggcctcctgagtggccaaagaccctgctgagatgacactgggccatggggtagagggccttgcaggcaaaggtgccactccgcagcaggtgcagtggaggccgaggcttggccatgaggagcacatcagtgaagaggaagaacatgcggggccgaggctccccatggggaggcaccactaacagccagccctggcgtaggaaccagcgccctgaggtcagcccctttgcctggcgtccactgagcagagcctggacacgccgaaggtgctggtcattcttctgtttctgaccaatagtatggactctctgggcagtctcacttatcagtcgggcagcccgtgtgagctgttgatggtcagggctgttgggacctgtgttttcagccaaagctacgacgagattctcatactgctggagccgttgcagaggcagagggagcaggtcctggagctgaaggcccccaaactcagggcggccttcctgaagccgtacaaacctccggaaacctttatttttctttagctgctcctgcagggtggtctgggacctctctgagttggcagcaaattggttatagagctccaagtggcggcagaagccctccagcccttggccccagcatcctccttccaggtagggaagcagctcctggctggcgccgtagatgagctcccaggagccaaacagggcctggcgctcaggtggtcgcagggtccccttggctttcaggatccccaaaaagtacgtggccaccagccccagctgttcttggtagcgccgctcggtctctagcagctcccgggcggtgcaggcgcgtttccgctcccagcgggcacgctgctcttgcaccgggcaccgcgaaccggggcaggagagctccatgccctggctgagggatcgacacttcc

SEQ ID NO: 15774 - RNA, 1252 nt, Homo sapiens
  source 1..1252: mol_type = other RNA
gctgggattacaggcatgagccactgtgcctggccgtgatttttaagagttggtcagatgatctggagtagcttggtccaggcaaacagaaagtgacctttgtcaaatcatgaagggttctgttttgttcagtactgaagattcctttgtactcttggctgtgacctatccctgaggtatcctgagttctggaatctataagattcctctagtttttctggctgctgatagcccaagtcagactgtggtaccagcgtgacagctcctcctggtctgtggacataagcagtagcttctcatgagggaaggacagactgagcaacccaccacaagggcctcctgagtggccaaagaccctgctgagatgacactgggccatggggtagagggccttgcaggcaaaggtgccactccgcagcaggtgcagtggaggccgaggcttggccatgaggagcacatcagtgaagaggaagaacatgcggggccgaggctccccatggggaggcaccactaacagccagccctggcgtaggaaccagcgccctgaggtcagcccctttgcctggcgtccactgagcagagcctggacacgccgaaggtgctggtcattcttctgtttctgaccaatagtatggactctctgggcagtctcacttatcagtcgggcagcccgtgtgagctgttgatggtcagggctgttgggacctgtgttttcagccaaagctacgacgagattctcatactgctggagccgttgcagaggcagagggagcaggtcctggagctgaaggcccccaaactcagggcggccttcctgaagccgtacaaacctccggaaacctttatttttctttagctgctcctgcagggtggtctgggacctctctgagttggcagcaaattggttatagagctccaagtggcggcagaagccctccagcccttggccccagcatcctccttccaggtagggaagcagctcctggctggcgccgtagatgagctcccaggagccaaacagggcctggcgctcaggtggtcgcagggtccccttggctttcaggatccccaaaaagtacgtggccaccagccccagctgttcttggtagcgccgctcggtctctagcagctcccgggcggtgcaggcgcgtttccgctcccagcgggcacgctgctcttgcaccgggcaccgcgaaccggggcaggagagctccatgccctggctgagggatcgacacttccggctgcagtc

SEQ ID NO: 15775 - RNA, 1123 nt, Homo sapiens
  source 1..1123: mol_type = other RNA
gctgggattacaggcatgagccactgtgcctggccgtgatttttaagagttggtcagatgatctggagtagcttggtccaggcaaacagaaagtgacctttgtcaaatcatgaagggttctgttttgttcagtactgaagattcctttgtactcttggctgtgacctatccctgaggtatcctgagttctggaatctataagattcctctagtttttctggctgctgatagcccaagtcagactgtggtaccagcgtgacagctcctcctggtctgtggacataagcagtagcttctcatgagggaaggacagactgagcaacccaccacaagggcctcctgagtggccaaagaccctgctgagatgacactgggccatggggtagagggccttgcaggcaaaggtgccactccgcagcaggtgcagtggaggccgaggcttggccatgaggagcacatcagtgaagaggaagaacatgcggggccgaggctccccatggggaggcaccactaacagccagccctggcgtaggaaccagcgccgtgtgagctgttgatggtcagggctgttgggacctgtgttttcagccaaagctacgacgagattctcatactgctggagccgttgcagaggcagagggagcaggtcctggagctgaaggcccccaaactcagggcggccttcctgaagccgtacaaacctccggaaacctttatttttctttagctgctcctgcagggtggtctgggacctctctgagttggcagcaaattggttatagagctccaagtggcggcagaagccctccagcccttggccccagcatcctccttccaggtagggaagcagctcctggctggcgccgtagatgagctcccaggagccaaacagggcctggcgctcaggtggtcgcagggtccccttggctttcaggatccccaaaaagtacgtggccaccagccccagctgttcttggtagcgccgctcggtctctagcagctcccgggcggtgcaggcgcgtttccgctcccagcgggcacgctgctcttgcaccgggcaccgcgaaccggggcaggagagctccatgccctggctgagggatcgacacttccggctgcagtc

SEQ ID NO: 15776 - RNA, 1238 nt, Homo sapiens
  source 1..1238: mol_type = other RNA
gctgggattacaggcatgagccactgtgcctggccgtgatttttaagagttggtcagatgatctggagtagcttggtccaggcaaacagaaagtgacctttgtcaaatcatgaagggttctgttttgttcagtactgaagattcctttgtactcttggctgtgacctatccctgaggtatcctgagttctggaatctataagattcctctagtttttctggctgctgatagcccaagtcagactgtggtaccagcgtgacagctcctcctggtctgtggacataagcagtagcttctcatgagggaaggacagcacaagggcctcctgagtggccaaagaccctgctgagatgacactgggccatggggtagagggccttgcaggcaaaggtgccactccgcagcaggtgcagtggaggccgaggcttggccatgaggagcacatcagtgaagaggaagaacatgcggggccgaggctccccatggggaggcaccactaacagccagccctggcgtaggaaccagcgccctgaggtcagcccctttgcctggcgtccactgagcagagcctggacacgccgaaggtgctggtcattcttctgtttctgaccaatagtatggactctctgggcagtctcacttatcagtcgggcagcccgtgtgagctgttgatggtcagggctgttgggacctgtgttttcagccaaagctacgacgagattctcatactgctggagccgttgcagaggcagagggagcaggtcctggagctgaaggcccccaaactcagggcggccttcctgaagccgtacaaacctccggaaacctttatttttctttagctgctcctgcagggtggtctgggacctctctgagttggcagcaaattggttatagagctccaagtggcggcagaagccctccagcccttggccccagcatcctccttccaggtagggaagcagctcctggctggcgccgtagatgagctcccaggagccaaacagggcctggcgctcaggtggtcgcagggtccccttggctttcaggatccccaaaaagtacgtggccaccagccccagctgttcttggtagcgccgctcggtctctagcagctcccgggcggtgcaggcgcgtttccgctcccagcgggcacgctgctcttgcaccgggcaccgcgaaccggggcaggagagctccatgccctggctgagggatcgacacttccggctgcagtc

SEQ ID NO: 15777 - RNA, 975 nt, Homo sapiens
  source 1..975: mol_type = other RNA
gctgggattacaggcatgagccactgtgcctggccgtgatttttaagagttggtcagatgatctggagtagcttggtccaggcaaacagaaagtgacctttgtcaaatcatgaagggttctgttttgttcagtactgaagattcctttgtactcttggctgtgacctatccctgaggtatcctgagttctggaatctataagattcctctagtttttctggctgctgatagcccaagtcagactgtggtaccagcgtgacagctcctcctggtctgtggacataagcagtagcttctcatgagggaaggacagcagacattgttggaggtcagaatcagaaaggaatacaggagaggaagcctccagcctgcgttgccgaggagcaagaacctacgtgtgagctgttgatggtcagggctgttgggacctgtgttttcagccaaagctacgacgagattctcatactgctggagccgttgcagaggcagagggagcaggtcctggagctgaaggcccccaaactcagggcggccttcctgaagccgtacaaacctccggaaacctttatttttctttagctgctcctgcagggtggtctgggacctctctgagttggcagcaaattggttatagagctccaagtggcggcagaagccctccagcccttggccccagcatcctccttccaggtagggaagcagctcctggctggcgccgtagatgagctcccaggagccaaacagggcctggcgctcaggtggtcgcagggtccccttggctttcaggatccccaaaaagtacgtggccaccagccccagctgttcttggtagcgccgctcggtctctagcagctcccgggcggtgcaggcgcgtttccgctcccagcgggcacgctgctcttgcaccgggcaccgcgaaccggggcaggagagctccatgccctggctgagggatcgacacttccggctgcagtc

SEQ ID NO: 15778 - RNA, 1329 nt, Homo sapiens
  source 1..1329: mol_type = other RNA
gctgggattacaggcatgagccactgtgcctggccgtgatttttaagagttggtcagatgatctggagtagcttggtccaggcaaacagaaagtgacctttgtcaaatcatgaagggttctgttttgttcagtactgaagattcctttgtactcttggctgtgacctatccctgaggtatcctgagttctggaatctataagattcctctagtttttctggctgctgatagcccaagtcagactgtggtaccagcgtgacagctcctcctggtctgtggacataagcagtagcttctcatgagggaaggacagctagagagagaccacctcttagcgcatggctcagaaaggtccaggctaaagctgaagcccttgctgtttccatggagactgagcaacccaccacaagggcctcctgagtggccaaagaccctgctgagatgacactgggccatggggtagagggccttgcaggcaaaggtgccactccgcagcaggtgcagtggaggccgaggcttggccatgaggagcacatcagtgaagaggaagaacatgcggggccgaggctccccatggggaggcaccactaacagccagccctggcgtaggaaccagcgccctgaggtcagcccctttgcctggcgtccactgagcagagcctggacacgccgaaggtgctggtcattcttctgtttctgaccaatagtatggactctctgggcagtctcacttatcagtcgggcagcccgtgtgagctgttgatggtcagggctgttgggacctgtgttttcagccaaagctacgacgagattctcatactgctggagccgttgcagaggcagagggagcaggtcctggagctgaaggcccccaaactcagggcggccttcctgaagccgtacaaacctccggaaacctttatttttctttagctgctcctgcagggtggtctgggacctctctgagttggcagcaaattggttatagagctccaagtggcggcagaagccctccagcccttggccccagcatcctccttccaggtagggaagcagctcctggctggcgccgtagatgagctcccaggagccaaacagggcctggcgctcaggtggtcgcagggtccccttggctttcaggatccccaaaaagtacgtggccaccagccccagctgttcttggtagcgccgctcggtctctagcagctcccgggcggtgcaggcgcgtttccgctcccagcgggcacgctgctcttgcaccgggcaccgcgaaccggggcaggagagctccatgccctggctgagggatcgacacttccggctgcagtc

SEQ ID NO: 15779 - RNA, 1200 nt, Homo sapiens
  source 1..1200: mol_type = other RNA
gctgggattacaggcatgagccactgtgcctggccgtgatttttaagagttggtcagatgatctggagtagcttggtccaggcaaacagaaagtgacctttgtcaaatcatgaagggttctgttttgttcagtactgaagattcctttgtactcttggctgtgacctatccctgaggtatcctgagttctggaatctataagattcctctagtttttctggctgctgatagcccaagtcagactgtggtaccagcgtgacagctcctcctggtctgtggacataagcagtagcttctcatgagggaaggacagctagagagagaccacctcttagcgcatggctcagaaaggtccaggctaaagctgaagcccttgctgtttccatggagactgagcaacccaccacaagggcctcctgagtggccaaagaccctgctgagatgacactgggccatggggtagagggccttgcaggcaaaggtgccactccgcagcaggtgcagtggaggccgaggcttggccatgaggagcacatcagtgaagaggaagaacatgcggggccgaggctccccatggggaggcaccactaacagccagccctggcgtaggaaccagcgccgtgtgagctgttgatggtcagggctgttgggacctgtgttttcagccaaagctacgacgagattctcatactgctggagccgttgcagaggcagagggagcaggtcctggagctgaaggcccccaaactcagggcggccttcctgaagccgtacaaacctccggaaacctttatttttctttagctgctcctgcagggtggtctgggacctctctgagttggcagcaaattggttatagagctccaagtggcggcagaagccctccagcccttggccccagcatcctccttccaggtagggaagcagctcctggctggcgccgtagatgagctcccaggagccaaacagggcctggcgctcaggtggtcgcagggtccccttggctttcaggatccccaaaaagtacgtggccaccagccccagctgttcttggtagcgccgctcggtctctagcagctcccgggcggtgcaggcgcgtttccgctcccagcgggcacgctgctcttgcaccgggcaccgcgaaccggggcaggagagctccatgccctggctgagggatcgacacttccggctgcagtc

SEQ ID NO: 15780 - RNA, 893 nt, Homo sapiens
  source 1..893: mol_type = other RNA
gctgggattacaggcatgagccactgtgcctggccgtgatttttaagagttggtcagatgatctggagtagcttggtccaggcaaacagaaagtgacctttgtcaaatcatgaagggttctgttttgttcagtactgaagattcctttgtactcttggctgtgacctatccctgaggtatcctgagttctggaatctataagattcctctagtttttctggctgctgatagcccaagtcagactgtggtaccagcgtgacagctcctcctggtctgtggacataagcagtagcttctcatgagggaaggacaggtgtgagctgttgatggtcagggctgttgggacctgtgttttcagccaaagctacgacgagattctcatactgctggagccgttgcagaggcagagggagcaggtcctggagctgaaggcccccaaactcagggcggccttcctgaagccgtacaaacctccggaaacctttatttttctttagctgctcctgcagggtggtctgggacctctctgagttggcagcaaattggttatagagctccaagtggcggcagaagccctccagcccttggccccagcatcctccttccaggtagggaagcagctcctggctggcgccgtagatgagctcccaggagccaaacagggcctggcgctcaggtggtcgcagggtccccttggctttcaggatccccaaaaagtacgtggccaccagccccagctgttcttggtagcgccgctcggtctctagcagctcccgggcggtgcaggcgcgtttccgctcccagcgggcacgctgctcttgcaccgggcaccgcgaaccggggcaggagagctccatgccctggctgagggatcgacacttccggctgcagtc

SEQ ID NO: 15781 - RNA, 3058 nt, Homo sapiens
  source 1..3058: mol_type = other RNA
gctgggattacaggcatgagccactgtgcctggccgttgttcaacaatttttaatgtcataaaagcctcatgcagacacaccgtaattcattgaaccccttttccactgacagggatcaggcttttctctgtttttcttgtgtatgcaatgctataaggacaattcctaaacattgcagtttgtggggatctcggataatttcctcaggatacattcctagaaataaaaattctgggccccagtacacaatcttaaggttttgccacctatcgtcaaactgctacggcctttctggagcgaaatttatattcccagtagccatgtgaaagaatgtttatttcatgttactcctcttgcacttaatactgccttaaaaaatatttgcacatttctctttgttacacatggcttctttttgctttgatctgtatactttttaaaaatattaccagtgagtcttcgatgattgcttcatgtttctgggaggtatttcgttcctgtgcgtttctggagttttcatcttttgaaaaaaatgactcataagagcccttcatattgttagatttttactaatgctttcttgctggtttaattttaggttaagtctttcctatccacaacagcaaaggccttgttctccctcgtgcaatctcaaaagctcaaaagtcaattaaaaaaattcaggcagaggcatacatggcacctataaaaatgatatcaactctatccctaaacaggggatgggacctggggaagccacttcccacatttaaatgttctatcaggaatttgtctagaagccagaagtttagaccttgctctgtggcctctctgattgaaatgcgaagtctgtttcctaagtaactcagaacttgttgtttgattttgatttttgacttttttatatgccccagtgggtcctggtcttgggagctcaactgggaagccgaaaggatacagcagagattttatatgccccagtgggtcctggtcttgggagctcaactgggaagccgaaaggacacagcagagaagggcaggccccctctcccaggccatttgactctcccaggccatttgaaaagacggtgcatcttcacataccattttttttgtgtcggccttctggggttgacagccctttcagtgagcacaaaacctcagcttgcatttattttgattttcgtaggtatcactgttgaaaagaaggaaagctgcctatcacagatgttaaacaaacaattgattgtttaatgactctgcaactgtggtttccaccctgggtgtggtgtagcgcgtgcacatttacacaacttccttggcatcgaagtcgcttagaagaatgcttcgatgcgagcagattttccgccgtgacaaaatacacagttgaggttttttctctctctctttcacagttcttgtctaccagcccctggcagaaatcaccatttcttcggcgaaggaatgctactttccaaaatcctttggcagaatctcctagagatttgtttttctgcttcctaatttagaaagtcttcaaagaaaaaaaaaacttgacaaattaatgtgagaagaaacgaactgtgatttaattttgcatttctttcatgaaaagtttatcatgtataaccaataaaattggataagatgattttgggggagaaaagtaaatgaaaatgtgttataccccaagatcagactgttcttttattctgagtcaataagtaacatgtgatacaaactcaagattttattaaaatcatttgtaagttaaattagcatatctcggtggtgaaggaagacttttaataaagcaaaataatgagttaggtgaatcaacagaaagagtgaaaagtgttaacagtgacatttaaatggttacatgattttaattattcttttgataataagcaaccttgtgatatctattcaagaaaagccagagcccactatggaattcgcagttgaataagagctttgttccctgcttttggtaatgttaaagaaacaaatggaaatggtttaaagaccttataacaatctcccacctagcaaaagaatctaaaaggtaaggtgggaagcattagaaagagagtgaaaagaaaaataaaaaaggcctcacacgcagcattgggtttatttgagagacagggcaagagagaatgaagtgttggagagagaaggtgctggaaggccagccgatgccaatcccttccttatctgttcttggctgccaggggtttccggctgatctttttcgatttgtcattattcttcttcggtggttctgggttggcctgcatgtgtctgccgtagaggctagttctgggggcagaacggtgaggcggttcccctgaatgtggagctctttaagctgggtaagctccccgatttccttaggcagcgagatcaggtcgttatccctaaggctgagtatctgcaactttgtgagcttcccaatatctggcggcaggatttcaaaatcgttgtcacttagatagagtgcacgcagggtggtcaggtagaagaagtttccaggaagagaattttcgctcaagttgttgtacgtcaagtccagaacctcaagagctggcagggagccgaagcctcgtggcaaagtgttcagcctgttcatgccaaggttcaggtgtttgagtttctgaaggctactgatctgtgtgggcagctcctcgatttggttattaaaaaagttgagcacctccaaattcttcagttctgcgatgttcggtggcaccattgttagcttgttatggctgaggaccagttgtgtgatatgggataaggtaaagaggccgttgacatccagcatgttggagatgccccggtcactcatgtccacctcgggctggttcttctcccggctctcctccaccaacttcttcagagacttggacatggtcacggaaggtagcccctaagacgatgggcgtgcaaccacaagcttcggcagaacgcactccagctgccctcactccctgcaacaccggcactgaacagcgaacacgccctgtctcggcgccccgcgcaggcgcacac

SEQ ID NO: 15782 - RNA, 3164 nt, Homo sapiens
  source 1..3164: mol_type = other RNA
gctgggattacaggcatgagccactgtgcctggccgttgttcaacaatttttaatgtcataaaagcctcatgcagacacaccgtaattcattgaaccccttttccactgacagggatcaggcttttctctgtttttcttgtgtatgcaatgctataaggacaattcctaaacattgcagtttgtggggatctcggataatttcctcaggatacattcctagaaataaaaattctgggccccagtacacaatcttaaggttttgccacctatcgtcaaactgctacggcctttctggagcgaaatttatattcccagtagccatgtgaaagaatgtttatttcatgttactcctcttgcacttaatactgccttaaaaaatatttgcacatttctctttgttacacatggcttctttttgctttgatctgtatactttttaaaaatattaccagtgagtcttcgatgattgcttcatgtttctgggaggtatttcgttcctgtgcgtttctggagttttcatcttttgaaaaaaatgactcataagagcccttcatattgttagatttttactaatgctttcttgctggtttaattttaggttaagtctttcctatccacaacagcaaaggccttgttctccctcgtgcaatctcaaaagctcaaaagtcaattaaaaaaattcaggcagaggcatacatggcacctataaaaatgatatcaactctatccctaaacaggggatgggacctggggaagccacttcccacatttaaatgttctatcaggaatttgtctagaagccagaagtttagaccttgctctgtggcctctctgattgaaatgcgaagtctgtttcctaagtaactcagaacttgttgtttgattttgatttttgacttttttatatgccccagtgggtcctggtcttgggagctcaactgggaagccgaaaggatacagcagagattttatatgccccagtgggtcctggtcttgggagctcaactgggaagccgaaaggacacagcagagaagggcaggccccctctcccaggccatttgactctcccaggccatttgaaaagacggtgcatcttcacataccattttttttgtgtcggccttctggggttgacagccctttcagtgagcacaaaacctcagcttgcatttattttgattttcgtaggtatcactgttgaaaagaaggaaagctgcctatcacagatgttaaacaaacaattgattgtttaatgactctgcaactgtggtttccaccctgggtgtggtgtagcgcgtgcacatttacacaacttccttggcatcgaagtcgcttagaagaatgcttcgatgcgagcagattttccgccgtgacaaaatacacagttgaggttttttctctctctctttcacagttcttgtctaccagcccctggcagaaatcaccatttcttcggcgaaggaatgctactttccaaaatcctttggcagaatctcctagagatttgtttttctgcttcctaatttagaaagtcttcaaagaaaaaaaaaacttgacaaattaatgtgagaagaaacgaactgtgatttaattttgcatttctttcatgaaaagtttatcatgtataaccaataaaattggataagatgattttgggggagaaaagtaaatgaaaatgtgttataccccaagatcagactgttcttttattctgagtcaataagtaacatgtgatacaaactcaagattttattaaaatcatttgtaagttaaattagcatatctcggtggtgaaggaagacttttaataaagcaaaataatgagttaggtgaatcaacagaaagagtgaaaagtgttaacagtgacatttaaatggttacatgattttaattattcttttgataataagcaaccttgtgatatctattcaagaaaagccagagcccactatggaattcgcagttgaataagagctttgttccctgcttttggtaatgttaaagaaacaaatggaaatggtttaaagaccttataacaatctcccacctagcaaaagaatctaaaaggtaaggtgggaagcattagaaagagagtgaaaagaaaaataaaaaaggcctcacacgcagcattgggtttatttgagagacagggcaagagagaatgaagtgttggagagagaaggtgctggaaggccagccgatgccaatcccttccttatctgttcttggctgccaggggtttccggctgatctttttcgatttgtcattattcttcttcggtggttctgggttggcctgcatgtgtctgccgtagaggtatttgtatgtctcagaacggatatactcaaaaacatgggacacgccaagctggaactggtctgcaatgggggtcacccagggattgttctctgctttgaatacctgcttctggccagttaaatccaagtttcctagttctgggggcagaacggtgaggcggttcccctgaatgtggagctctttaagctgggtaagctccccgatttccttaggcagcgagatcaggtcgttatccctaaggctgagtatctgcaactttgtgagcttcccaatatctggcggcaggatttcaaaatcgttgtcacttagatagagtgcacgcagggtggtcaggtagaagaagtttccaggaagagaattttcgctcaagttgttgtacgtcaagtccagaacctcaagagctggcagggagccgaagcctcgtggcaaagtgttcagcctgttcatgccaaggttcaggtgtttgagtttctgaaggctactgatctgtgtgggcagctcctcgatttggttattaaaaaagttgagcacctccaaattcttcagttctgcgatgttcggtggcaccattgttagcttgttatggctgaggaccagttgtgtgatatgggataaggtaaagaggccgttgacatccagcatgttggagatgccccggtcactcatgtccacctcgggctggttcttctcccggctctcctccaccaacttcttcagagacttggacatggtcacggaaggtagcccctaagacgatgggcgtgcaaccacaagcttcggcagaacgcactccagctgccctcactccctgcaacaccggcactgaacagcgaacacgccct

SEQ ID NO: 15783 - RNA, 3052 nt, Homo sapiens
  source 1..3052: mol_type = other RNA
gctgggattacaggcatgagccactgtgcctggccgttgttcaacaatttttaatgtcataaaagcctcatgcagacacaccgtaattcattgaaccccttttccactgacagggatcaggcttttctctgtttttcttgtgtatgcaatgctataaggacaattcctaaacattgcagtttgtggggatctcggataatttcctcaggatacattcctagaaataaaaattctgggccccagtacacaatcttaaggttttgccacctatcgtcaaactgctacggcctttctggagcgaaatttatattcccagtagccatgtgaaagaatgtttatttcatgttactcctcttgcacttaatactgccttaaaaaatatttgcacatttctctttgttacacatggcttctttttgctttgatctgtatactttttaaaaatattaccagtgagtcttcgatgattgcttcatgtttctgggaggtatttcgttcctgtgcgtttctggagttttcatcttttgaaaaaaatgactcataagagcccttcatattgttagatttttactaatgctttcttgctggtttaattttaggttaagtctttcctatccacaacagcaaaggccttgttctccctcgtgcaatctcaaaagctcaaaagtcaattaaaaaaattcaggcagaggcatacatggcacctataaaaatgatatcaactctatccctaaacaggggatgggacctggggaagccacttcccacatttaaatgttctatcaggaatttgtctagaagccagaagtttagaccttgctctgtggcctctctgattgaaatgcgaagtctgtttcctaagtaactcagaacttgttgtttgattttgatttttgacttttttatatgccccagtgggtcctggtcttgggagctcaactgggaagccgaaaggatacagcagagattttatatgccccagtgggtcctggtcttgggagctcaactgggaagccgaaaggacacagcagagaagggcaggccccctctcccaggccatttgactctcccaggccatttgaaaagacggtgcatcttcacataccattttttttgtgtcggccttctggggttgacagccctttcagtgagcacaaaacctcagcttgcatttattttgattttcgtaggtatcactgttgaaaagaaggaaagctgcctatcacagatgttaaacaaacaattgattgtttaatgactctgcaactgtggtttccaccctgggtgtggtgtagcgcgtgcacatttacacaacttccttggcatcgaagtcgcttagaagaatgcttcgatgcgagcagattttccgccgtgacaaaatacacagttgaggttttttctctctctctttcacagttcttgtctaccagcccctggcagaaatcaccatttcttcggcgaaggaatgctactttccaaaatcctttggcagaatctcctagagatttgtttttctgcttcctaatttagaaagtcttcaaagaaaaaaaaaacttgacaaattaatgtgagaagaaacgaactgtgatttaattttgcatttctttcatgaaaagtttatcatgtataaccaataaaattggataagatgattttgggggagaaaagtaaatgaaaatgtgttataccccaagatcagactgttcttttattctgagtcaataagtaacatgtgatacaaactcaagattttattaaaatcatttgtaagttaaattagcatatctcggtggtgaaggaagacttttaataaagcaaaataatgagttaggtgaatcaacagaaagagtgaaaagtgttaacagtgacatttaaatggttacatgattttaattattcttttgataataagcaaccttgtgatatctattcaagaaaagccagagcccactatggaattcgcagttgaataagagctttgttccctgcttttggtaatgttaaagaaacaaatggaaatggtttaaagaccttataacaatctcccacctagcaaaagaatctaaaaggtaaggtgggaagcattagaaagagagtgaaaagaaaaataaaaaaggcctcacacgcagcattgggtttatttgagagacagggcaagagagaatgaagtgttggagagagaaggtgctggaaggccagccgatgccaatcccttccttatctgttcttggctgccaggggtttccggctgatctttttcgatttgtcattattcttcttcggtggttctgggttggcctgcatgtgtctgccgtagaggtatttgtatgtctcagaacggatatactcaaaaacatgggacacgccaagctggaactggtctgcaatgggggtcacccagggattgttctctgctttgaatacctgcttctggccagttaaatccaagtttcctagttctgggggcagaacggtgaggcggttcccctgaatgtggagctctttaagctgggtaagctccccgatttccttaggcagcgagatcaggtcgttatccctaaggctgagtatctgcaactttgtgagcttcccaatatctggcggcaggatttcaaaatcgttgtcacttagatagagtgcacgcagggtggtcaggtagaagaagtttccaggaagagaattttcgctcaagttgttgtacgtcaagtccagaacctcaagagctggcagggagccgaagcctcgtggcaaagtgttcagcctgttcatgccaaggttcaggtgtttgagtttctgaaggctactgatctgtgtgggcagctcctcgatttggttattaaaaaagttgagcacctccaaattcttcagttctgcgatgttcggtggcaccattgttagcttgttatggctgaggaccagttgtgtgatatgggataaggtaacacggaaggtagcccctaagacgatgggcgtgcaaccacaagcttcggcagaacgcactccagctgccctcactccctgcaacaccggcactgaacagcgaacacgccct

SEQ ID NO: 15784 - RNA, 62 nt, Homo sapiens
  source 1..62: mol_type = other RNA
gctgggattacaggcatgagccactgtgcctggcctatactttttatttttattattattat

SEQ ID NO: 15785 - RNA, 310 nt, Homo sapiens
  source 1..310: mol_type = other RNA
gctgggattacaggcatgagccactgtgcctggcctcacttttcaatataggattgttgattttgaagacaattgaggccaagcatcgtgggtcatgcctgtaatgccagcattttgggaggcagaggcaggcagatcacctgaggtcaggagtgcaagaccagcctgaccaacatggtgaaacctcatctccattaaaaatacaaaaactcactttgggaggccaaggcgggcggatcaagaggtcaggagatcgagaccaccctggctaacacggtgaaaccccgtctctactaaaaatacaaaaaat

SEQ ID NO: 15786 - RNA, 4108 nt, Homo sapiens
  source 1..4108: mol_type = other RNA
gctgggattacaggcatgagccactgtgcctggcctgaatttttaataagtaagttataggtatcatgacatctcacaccaaaatacttgagcatacatcatcacggaggattctctctgaagtgttgaaggttgtgtgtatcgtccgcattgctgaaggaaggcttcaaggtgttgtgcatatgagctctgtcatttctcaactgactgagtccagttgtttccaagcagaaattcatcaggacattaccatcactcatgaggagaaagtgttgggtggaaccaaagacggtcttagctgtatttgaaacatttctgattcttctttgctattccgcgagctcaggaggctggaaactctaagaactgttctgggtgcggcagcccaggtagagaaggagcccagtaaacgctcagagattcacccacagggcccttcccagagtggaggccccagcgctagggagcttcggcctcaaacactttgtctcctgggttctgaagccttatctttgtcaccttgatttgattcattaatatacagacattgcttctctcccctacttgattaggagccccttgaggacagaatgtgtttctctctttatttctgtaaccagcatagtgtttggtacattgttgaggctcgacaaatattcctgaatcaataaatgactcaactaatcagcccatatgtgtctatagggcctaaatgaggtgagtgtggagaagcaattatgtggaaccaattgtgcaggcgctgagcaggcccagcatggggcctggggggccgtctttggtggctggtcctgcctggtcctgctccactgcctcggtctcattccaagggaaatatttgttctgtgagcaaataaaatgtgaatatgttctaatctgttgcaaggatacacagagctgccttcagcctggtgcttagatctctgagggcacttcaaagaactgcaaaaataaaatgtcctctgtggagcgggaaaaatggagctctttcctgcccagagagaagggcaaatgaagactggatgacaagtttcccgcttgaagataacgtaaatcaaatctgctctgggcccatcaggaccccagacatgagaggtgattacagacttctcttcctatcatgctatgtacttagaagtgctgaacctgccgtttgaaaacacacagacacacacaccagaaatctttacttcatgcccatgtttaactaatgaaggagaagtcccagctcccagcaatgcgtgtgttgaaccacgtcttgtctgcctcgctggccagctgaactagccttttgcccactcaagtaccacacaccgtggaccctgtgtgcctacattttaacaaacatgcagaatggatgggagaagtgaggaagagaaaaacaaaaattcccagtcgcagaaaattaggaggatatctttgtattttgtttgtctcctactaaggaattcttagaagttcagaaccttccataataagctgtcatcggatacacttgtttccgcatagggcctcgggtttgattgcagggtttttaagcttctggcagaggaatgcaatgtttcaacgttgccttagcccaaccccgtcccttttcacaggctggggcaaaaaaaaaaaaaaaaaaaaaatagtgttgaactgtccagtgtgcaaattaaatcatttattaaaggctgaagagagagggtttaagatccccacagtggattctgaaactataacccaggattccctctttacatccatgttctgtacgtgcaagtctcttgtgttgcgctgtcctgaggtcaggcaggcctattttgaattctgggttaagaacaagcctcagccatcccttagggcacagccttagctgccatttactgatcctcccttggtgtttaaatcctctcaacaacaaactgcaggtgagaaatattagtgtcattatcagcctcattttgttagtggggaatctgaggctcagagacatcaagcaacctgcccaatatggcccagctggtattagaattctgctttgccaactccaacactcgtcctgtcaccccggtgaactcaccaaggaagtcagcctgcctggaacttcacgaatactattcctactagtttatcattcaaagtaacctctattctctatttcattagatcgcccatttttaacatgtgtaatttaatttaaaaatcacacaatactagcccagtccattcaaaaggctttttgaaaacctctgtttcctttgaaaatggattgttatctatggccataccaccctgaacaaacccgacctcatgtgaaaatggattgtagtttaggttcctccatttcaaagtggaattgcaagacctccctaacgtgtttacaacattcctgtgctgagtgttatcccttctcccaggagccagattgacagtctctagcgcagccctctctttggctgacagctgtcattcataatggcaagggggcagtcctatccccatctaaaataggcaacagaatgtagccagatcgcctactgtcatacctatactaaaacacacacaaacacacacacacacacacacacacacacacaaagatattcacggtagtgttttttttaacctcaaaaaattggaaacagcctaatactcaatcaacattagggaaacaagcaaatcatattatagctataagaagacatactaagcaaactttaaaaattgagtttttgaagaatgtttaataacctagagccactcctatgacataatactaggaaaaaatacaaagctttttatcttttaaaatctccattatgtaaaacagcaagaaaaaaagacagggaggaaatatgcttaaatgttaacagtattcatttctagaatgatggatgtttagtttatttgtaattattttttatatttccctaactgtatacaatggatatagaatgattttacaatttaaaatgtctttgtaactcccaattagggtgaatggagaagattgattttaaaacttaacaaaaacaaatgcttttggagaaactgtaacaaatgagattattaaatatctgaaacctctctgattggaattaggccataagtttaattttttttaagtatcatgacagataggcatgcctgccagctgaaagaactattttacttcccacggcactcccttacaaataatgtaccaagtctttttaaaacaacaaatgtaacagcctacaggattctgttacttgtttaccctggacctgggctcaaaatggcttgaatctatctccaccattcaagatcagccctgatgaacaaatccctggtgtgcctagaaggagggagggtggggaagaagtcaggggaggagcaaatatgagcctccccacccccccactcacacctggtgtggagctttgtcaattactcactgaaggaatgtaaaactctgttcttcctaccggatccaagctagcagaggcagaaagcagcagcagcaggacatgctgggttgattccaagacactgaagagtgttgatagcccagacagcttccctgttcttccttgtgaacccagtcctgttcctctgagctttggggtgttctgagccgggacaagaaggcatctgaagaatgctttttctgatcccccatctcttcagccaggtctgtgctctctttctctcacctctctgctatgatgcacttcaacctacccttcaccctcatcaggtttgtcgttcccaaatttcccccttccatttgtcactcctttactctacaacttaccatggcttgaagaatcagacccaaattcctcagatccccaatacacagcccctacccaacttcctccaaactcacctccctcacccccaccccatcccacctactcccaccctaaccccagcacccaacccagctctccctgcagactgaacttcagtggcactccgaagttggaaagaaatgttccttcactaaaatagaatagtggaagcttgtccaaattatgctcaaagatacaattttctcaatgttaagtttttcccatcaatttttgttaaacctttggcactcacagctctgcctatctct

SEQ ID NO: 15787 - RNA, 4872 nt, Homo sapiens
  source 1..4872: mol_type = other RNA
gctgggattacaggcatgagccactgtgcctggcctgtgacatcagttttaagagtttcaggattttgtgtacattcatgatggttactgaaacatacatttccaggtacaatttcaaagtcaaaaggcaatgcttaaagcttctggtattgattgccagagatggtatgtatttattcatgtcttaccagcagcattagagtcccaatgtccctgaatccctgtctgttttataaggaaaagtgtcatctcaactcttgctttaatatacattttaactgtagtgaggttgaacatttattgttcattggcacttattttgtgatttccctacttaagtagcattttttttctattggaactttcttatggggagagagtatactgaagtggctccacagtcaggttgtgggttcaaagtctgacctccccactttgtagatatatgacctttagccttcatttcctcatctgctacatacgtgctgagaaataacaataataagtatatacaaagcccttagcaagtatctattacatttacttttttcctttttttttggtttggagacagggtcttgctctcccaggctggagtgcagtggtgtgatcttgcctcactgaagcctcgacttccagggctcaagcgaacctctcacctcagcctcccaaatacttgggtctacaggcatgcactaccacgtctggcaaattctgtttattttttgtagagatggggtctcactatgctgcccaggctcggcttgaactcctagactcaagcaatcctccagccttggcctcccaaagtgctggcattataggtgtgagccactgtgcttggtctatctattacattgctttctgacatacagtagagctttcttatataaagagtatttccgttttacaattcctactttacgtcctaccttttcagtttgttcaggtctttatctatggaaaaggagaaaaacaagagttgagtagctcttaccacgtattttaatctcttacatcttttccaaataatcccatccattttttccatattctctccctaaacatgggcatttaggcctcctgctgttcttactggttagcacatgtccactgatgcacgccccaataagagcattacttctctttgcttctttttatcctcatgaaaattctttttctatgcacatgattctagatttccatacagatttgtttttggtgtggtatgttattcttctgacctattaggtcttttgaatatgtctttgtgttgctggttaacctgtacaacattccttcttacactaagcatcagtctaaatattctcttcctgctaggcccctcagaaaagggaagtcttgactgactgtgaccattagtttcagttgtcacttccttttagcattgtctttaataaaatttgcaaaagatggttgggcgccatggctcacgcctgtaatcccagcactttggggggccgaggcgggcggatcacctgagatcgagaattcgagaccagcctgaccaacatggagaaaccctgtctttcctaaaaatacaaaattagccagctgtggtggtgcatgcctgtaatcccagctactcagaaggctgaggcaggagaatcgcttgaacccaggaggcagagtttgcggtgagccaagatcgtgccattgcactccagcctggacaagagcgaactccatctcaaaaaaaaaaaaaaaaaaaaaaaaattgcaaaagatattgtgaaatactggtgacataagacaaaactgaacatgtgcgaggtgcccaaagaatgtcacagacccagcaactgacaaatattttttgagcaccaaagcccaagggaatgtactaggaattgtgggcgtatagccccagaaacaaatgatatggcagcttctgatccagagcgttgggaattttaagaaacctgacagcagctctgatattgtctttagaatcaaaggagaatagagtcttaacactctagcagactcttgaggtataggctgggctctttctcaccctcattcccaccaccaccctcatggaagttctaggatagcctacaggttgggcaaggaaaccacatatttgccctttccctggggtcacataaaccaagacaaagctcttgactaccctgtggcccaagggctccaggttttgtctattaacaggaacttctccattggcactgcttaagagtctggccagacccagacttctctgacagacaagacctcactacaacaggaactcaaggaatgctccacactttgtttctggcctttggctactgttctttactggggtaccacttccctagagtaccaccttggctaactcctcctcatccttcaggccatttcccccatttccttatccaaggctgagtcaggtgctccttaaggtcacataggagcattccactttcactgcctgtctggctgccttgcccattagactgtagagactacagtcttgttttccactgtattcctagttcctgggacaaagtaggtactcaaaaaataacctttgggtaaattatattctttcttctcatgcctatctaattcctggcctgccctgggctcaacaaatcattgatgaagccatttccccacctttcctgctgctctgtcactgttctttattgggtcagttttttttttttttttagttcctgagacgaagtgcctcacacagtccacaccagccccataacctggcacactaacaatcagatgcagtgacagagcctgggttgctatattcatgacactttcatacaaaatgaggtttcaatgttacattcccacttttcgtatttcctgagtattcctaataagagaagagctggaagtaatgattcttctgtattctgttctgattagtcacaggaaaagctttcaagggacactttacattagcactgggaaatgctgcacaaagcaagctagactcaagacctagtattttataacctttatggagttttgctccaaagtaaactcttttgactaacaaacttaaaaatctgactgaagtatttacactattcacagtattcacaaattactttatagtgtggactctttgatggcgcataaggaccgatctgtgcctgaaagccttcccacattcattacatatataagcttcatccccagaatgaattctctgatgctgaacaagggctgagctccttttgaaagttttgccacattcattacactgataaggttcctccccactatgaattctctgatgtctgataaggtttgagctcaaactgaaagcttttccacattcactacattcatagggtttctctccactatgtattctctgatgagtaatcagctctgagctctgcctgaaagcttttccacattcattacattcatagggtctctctcctgtgtgaattcgctgatgtctaatgagttttgagctctggctaaaggttttcccacattcattacactcataaggtttctcaccagtgtgaattctttgatgtataatgagatatgaactttgactgaatgctttgccacactcattacatttacaagctttctcaccagtatggattttccgatgtctaatgagggctgagctctgattgaaagctttcccacattcactacattcatatgctttctcaccactatgaattctctgatgaataataagataggacctcaaactaaaggccttcccacactggttacatttatagggcttttctccagtatggattctctgatgttgtgttagagaggaatgctgcttgaagctgtgcccacatacatcacatctataaggtctctcttctggaggaactttctgacacattatagagtctgtagttagaatcaagcatctttcagcctcatcataaaggtctctctttcctagagatttgtttgtgaagatcacttgactaaaactgcccccttgggaaggagatcttagtttctcccctgtagcacttccttgcttccacactaaattgctttcatgctcactaattcctcgaaatgaaggttcctgagggagtccctgtgatttttcttctgagatgccctcttttgttgctgtttcactgttctcacaatacaggagggctgacagcaattcatgaggggtgaatacaaagccgctaaagcgagcacctctggtttagaataataaaggtgatgctcacatgtggcaagtttgtcaagtgcaattaattctgcattctcaaaaacagaggcctaagtgtcaagagtttccagatgatttcccattcctcaccacttttaggggaaaggcatggtttccaggatttcagctgtgtctttaagggctggaggtggatgtctgttgactcttgggatgctctgagacatgttaaatccttccatggcactgctggtccctgtggactagctgggaccgcgaagcccaggagcggccaggaaatgagccacccaccccgagctgcaagccacaaagaccggaagtgcgcgtacgcagtgttccgctctcgcgcccttcgggtcctccgccgccccgccccttgctctgaggtagccaatcagagccgcgggctctacagtttccaccgccttctcccggtagccgctagcccggcggaatctccaaggccaggggagggtgcgctaggagtcaggggtccttgtgagcggcggcacctggagggtcccgcatctcgcctgggccgttcccaccctggctttctcctggcaccacccatcattgttggtctcaagtaattcccgaatctcactcccagttttccattaaaatattcagattttcggccgggcgcggtggccgag

SEQ ID NO: 15788 - RNA, 5015 nt, Homo sapiens
  source 1..5015: mol_type = other RNA
gctgggattacaggcatgagccactgtgcctggcctgtgacatcagttttaagagtttcaggattttgtgtacattcatgatggttactgaaacatacatttccaggtacaatttcaaagtcaaaaggcaatgcttaaagcttctggtattgattgccagagatggtatgtatttattcatgtcttaccagcagcattagagtcccaatgtccctgaatccctgtctgttttataaggaaaagtgtcatctcaactcttgctttaatatacattttaactgtagtgaggttgaacatttattgttcattggcacttattttgtgatttccctacttaagtagcattttttttctattggaactttcttatggggagagagtatactgaagtggctccacagtcaggttgtgggttcaaagtctgacctccccactttgtagatatatgacctttagccttcatttcctcatctgctacatacgtgctgagaaataacaataataagtatatacaaagcccttagcaagtatctattacatttacttttttcctttttttttggtttggagacagggtcttgctctcccaggctggagtgcagtggtgtgatcttgcctcactgaagcctcgacttccagggctcaagcgaacctctcacctcagcctcccaaatacttgggtctacaggcatgcactaccacgtctggcaaattctgtttattttttgtagagatggggtctcactatgctgcccaggctcggcttgaactcctagactcaagcaatcctccagccttggcctcccaaagtgctggcattataggtgtgagccactgtgcttggtctatctattacattgctttctgacatacagtagagctttcttatataaagagtatttccgttttacaattcctactttacgtcctaccttttcagtttgttcaggtctttatctatggaaaaggagaaaaacaagagttgagtagctcttaccacgtattttaatctcttacatcttttccaaataatcccatccattttttccatattctctccctaaacatgggcatttaggcctcctgctgttcttactggttagcacatgtccactgatgcacgccccaataagagcattacttctctttgcttctttttatcctcatgaaaattctttttctatgcacatgattctagatttccatacagatttgtttttggtgtggtatgttattcttctgacctattaggtcttttgaatatgtctttgtgttgctggttaacctgtacaacattccttcttacactaagcatcagtctaaatattctcttcctgctaggcccctcagaaaagggaagtcttgactgactgtgaccattagtttcagttgtcacttccttttagcattgtctttaataaaatttgcaaaagatggttgggcgccatggctcacgcctgtaatcccagcactttggggggccgaggcgggcggatcacctgagatcgagaattcgagaccagcctgaccaacatggagaaaccctgtctttcctaaaaatacaaaattagccagctgtggtggtgcatgcctgtaatcccagctactcagaaggctgaggcaggagaatcgcttgaacccaggaggcagagtttgcggtgagccaagatcgtgccattgcactccagcctggacaagagcgaactccatctcaaaaaaaaaaaaaaaaaaaaaaaaattgcaaaagatattgtgaaatactggtgacataagacaaaactgaacatgtgcgaggtgcccaaagaatgtcacagacccagcaactgacaaatattttttgagcaccaaagcccaagggaatgtactaggaattgtgggcgtatagccccagaaacaaatgatatggcagcttctgatccagagcgttgggaattttaagaaacctgacagcagctctgatattgtctttagaatcaaaggagaatagagtcttaacactctagcagactcttgaggtataggctgggctctttctcaccctcattcccaccaccaccctcatggaagttctaggatagcctacaggttgggcaaggaaaccacatatttgccctttccctggggtcacataaaccaagacaaagctcttgactaccctgtggcccaagggctccaggttttgtctattaacaggaacttctccattggcactgcttaagagtctggccagacccagacttctctgacagacaagacctcactacaacaggaactcaaggaatgctccacactttgtttctggcctttggctactgttctttactggggtaccacttccctagagtaccaccttggctaactcctcctcatccttcaggccatttcccccatttccttatccaaggctgagtcaggtgctccttaaggtcacataggagcattccactttcactgcctgtctggctgccttgcccattagactgtagagactacagtcttgttttccactgtattcctagttcctgggacaaagtaggtactcaaaaaataacctttgggtaaattatattctttcttctcatgcctatctaattcctggcctgccctgggctcaacaaatcattgatgaagccatttccccacctttcctgctgctctgtcactgttctttattgggtcagttttttttttttttttagttcctgagacgaagtgcctcacacagtccacaccagccccataacctggcacactaacaatcagatgcagtgacagagcctgggttgctatattcatgacactttcatacaaaatgaggtttcaatgttacattcccacttttcgtatttcctgagtattcctaataagagaagagctggaagtaatgattcttctgtattctgttctgattagtcacaggaaaagctttcaagggacactttacattagcactgggaaatgctgcacaaagcaagctagactcaagacctagtattttataacctttatggagttttgctccaaagtaaactcttttgactaacaaacttaaaaatctgactgaagtatttacactattcacagtattcacaaattactttatagtgtggactctttgatggcgcataaggaccgatctgtgcctgaaagccttcccacattcattacatatataagcttcatccccagaatgaattctctgatgctgaacaagggctgagctccttttgaaagttttgccacattcattacactgataaggttcctccccactatgaattctctgatgtctgataaggtttgagctcaaactgaaagcttttccacattcactacattcatagggtttctctccactatgtattctctgatgagtaatcagctctgagctctgcctgaaagcttttccacattcattacattcatagggtctctctcctgtgtgaattcgctgatgtctaatgagttttgagctctggctaaaggttttcccacattcattacactcataaggtttctcaccagtgtgaattctttgatgtataatgagatatgaactttgactgaatgctttgccacactcattacatttacaagctttctcaccagtatggattttccgatgtctaatgagggctgagctctgattgaaagctttcccacattcactacattcatatgctttctcaccactatgaattctctgatgaataataagataggacctcaaactaaaggccttcccacactggttacatttatagggcttttctccagtatggattctctgatgttgtgttagagaggaatgctgcttgaagctgtgcccacatacatcacatctataaggtctctcttctggaggaactttctgacacattatagagtctgtagttagaatcaagcatctttcagcctcatcataaaggtctctctttcctagagatttgtttgtgaagatcacttgactaaaactgcccccttgggaaggagatcttagtttctcccctgtagcacttccttgcttccacactaaattgctttcatgctcactaattcctcgaaatgaaggttcctgagggagtccctgtgatttttcttctgagatgccctcttttgttgctgtttcactgttctcacaatacaggagggctgacagcaattcatgaggggtgaatacaaagccgctaaagcgagcacctctggtttagaataataaaggtgatgctcacatgtggcaagtttgtcaagtgcaattaattctgcattctcaaaaacagaggcctaagtgtcaagagtttccagatgatttcccattcctcaccacttttaggggaaaggcatggtttccaggatttcagctgtgtctttaagggctggaggtggatgtctgttgactcttgggatgctctgagacatgttaaatccttccatggcactgctggtccctgtggactagctgggacctgctgccctgggtcatcaaactccctctctaaatcctccaacagggtcacagcttcctcgccgctttctggattatgttgctgaacccagatctgcagctcctcaggcagaatgctcaggaactgctccagtaccagcagttctaagatctgctcctttgtgtgcaactctggcattagccactgatagcaaagttcctggagtcggctcagagcctcccggggcccaggtgtctcctggtagcaaaattttctgaattgctgacgaaacaattcttggcaggattgagtactcccattctgcttaaatttctcatcccaggaaaagttatcttctactttcactagtattagttcttgttccggaggatcctgaggtatcagggttgaaatcactccagattccacagccattcttggctgaaacagcttagcaaaaagctcagtacaactggttctgtgcttgcgaaggagtgtgagtaatctcttctttccgcgaagcccaggagcggccaggaaatgagccacccaccccgagctgcaagccac

SEQ ID NO: 15789 - RNA, 4947 nt, Homo sapiens
  source 1..4947: mol_type = other RNA
gctgggattacaggcatgagccactgtgcctggcctgtgacatcagttttaagagtttcaggattttgtgtacattcatgatggttactgaaacatacatttccaggtacaatttcaaagtcaaaaggcaatgcttaaagcttctggtattgattgccagagatggtatgtatttattcatgtcttaccagcagcattagagtcccaatgtccctgaatccctgtctgttttataaggaaaagtgtcatctcaactcttgctttaatatacattttaactgtagtgaggttgaacatttattgttcattggcacttattttgtgatttccctacttaagtagcattttttttctattggaactttcttatggggagagagtatactgaagtggctccacagtcaggttgtgggttcaaagtctgacctccccactttgtagatatatgacctttagccttcatttcctcatctgctacatacgtgctgagaaataacaataataagtatatacaaagcccttagcaagtatctattacatttacttttttcctttttttttggtttggagacagggtcttgctctcccaggctggagtgcagtggtgtgatcttgcctcactgaagcctcgacttccagggctcaagcgaacctctcacctcagcctcccaaatacttgggtctacaggcatgcactaccacgtctggcaaattctgtttattttttgtagagatggggtctcactatgctgcccaggctcggcttgaactcctagactcaagcaatcctccagccttggcctcccaaagtgctggcattataggtgtgagccactgtgcttggtctatctattacattgctttctgacatacagtagagctttcttatataaagagtatttccgttttacaattcctactttacgtcctaccttttcagtttgttcaggtctttatctatggaaaaggagaaaaacaagagttgagtagctcttaccacgtattttaatctcttacatcttttccaaataatcccatccattttttccatattctctccctaaacatgggcatttaggcctcctgctgttcttactggttagcacatgtccactgatgcacgccccaataagagcattacttctctttgcttctttttatcctcatgaaaattctttttctatgcacatgattctagatttccatacagatttgtttttggtgtggtatgttattcttctgacctattaggtcttttgaatatgtctttgtgttgctggttaacctgtacaacattccttcttacactaagcatcagtctaaatattctcttcctgctaggcccctcagaaaagggaagtcttgactgactgtgaccattagtttcagttgtcacttccttttagcattgtctttaataaaatttgcaaaagatggttgggcgccatggctcacgcctgtaatcccagcactttggggggccgaggcgggcggatcacctgagatcgagaattcgagaccagcctgaccaacatggagaaaccctgtctttcctaaaaatacaaaattagccagctgtggtggtgcatgcctgtaatcccagctactcagaaggctgaggcaggagaatcgcttgaacccaggaggcagagtttgcggtgagccaagatcgtgccattgcactccagcctggacaagagcgaactccatctcaaaaaaaaaaaaaaaaaaaaaaaaattgcaaaagatattgtgaaatactggtgacataagacaaaactgaacatgtgcgaggtgcccaaagaatgtcacagacccagcaactgacaaatattttttgagcaccaaagcccaagggaatgtactaggaattgtgggcgtatagccccagaaacaaatgatatggcagcttctgatccagagcgttgggaattttaagaaacctgacagcagctctgatattgtctttagaatcaaaggagaatagagtcttaacactctagcagactcttgaggtataggctgggctctttctcaccctcattcccaccaccaccctcatggaagttctaggatagcctacaggttgggcaaggaaaccacatatttgccctttccctggggtcacataaaccaagacaaagctcttgactaccctgtggcccaagggctccaggttttgtctattaacaggaacttctccattggcactgcttaagagtctggccagacccagacttctctgacagacaagacctcactacaacaggaactcaaggaatgctccacactttgtttctggcctttggctactgttctttactggggtaccacttccctagagtaccaccttggctaactcctcctcatccttcaggccatttcccccatttccttatccaaggctgagtcaggtgctccttaaggtcacataggagcattccactttcactgcctgtctggctgccttgcccattagactgtagagactacagtcttgttttccactgtattcctagttcctgggacaaagtaggtactcaaaaaataacctttgggtaaattatattctttcttctcatgcctatctaattcctggcctgccctgggctcaacaaatcattgatgaagccatttccccacctttcctgctgctctgtcactgttctttattgggtcagttttttttttttttttagttcctgagacgaagtgcctcacacagtccacaccagccccataacctggcacactaacaatcagatgcagtgacagagcctgggttgctatattcatgacactttcatacaaaatgaggtttcaatgttacattcccacttttcgtatttcctgagtattcctaataagagaagagctggaagtaatgattcttctgtattctgttctgattagtcacaggaaaagctttcaagggacactttacattagcactgggaaatgctgcacaaagcaagctagactcaagacctagtattttataacctttatggagttttgctccaaagtaaactcttttgactaacaaacttaaaaatctgactgaagtatttacactattcacagtattcacaaattactttatagtgtggactctttgatggcgcataaggaccgatctgtgcctgaaagccttcccacattcattacatatataagcttcatccccagaatgaattctctgatgctgaacaagggctgagctccttttgaaagttttgccacattcattacactgataaggttcctccccactatgaattctctgatgtctgataaggtttgagctcaaactgaaagcttttccacattcactacattcatagggtttctctccactatgtattctctgatgagtaatcagctctgagctctgcctgaaagcttttccacattcattacattcatagggtctctctcctgtgtgaattcgctgatgtctaatgagttttgagctctggctaaaggttttcccacattcattacactcataaggtttctcaccagtgtgaattctttgatgtataatgagatatgaactttgactgaatgctttgccacactcattacatttacaagctttctcaccagtatggattttccgatgtctaatgagggctgagctctgattgaaagctttcccacattcactacattcatatgctttctcaccactatgaattctctgatgaataataagataggacctcaaactaaaggccttcccacactggttacatttatagggcttttctccagtatggattctctgatgttgtgttagagaggaatgctgcttgaagctgtgcccacatacatcacatctataaggtctctcttctggaggaactttctgacacattatagagtctgtagttagaatcaagcatctttcagcctcatcataaaggtctctctttcctagagatttgtttgtgaagatcacttgactaaaactgcccccttgggaaggagatcttagtttctcccctgtagcacttccttgcttccacactaaattgctttcatgctcactaattcctcgaaatgaaggttcctgagggagtccctgtgatttttcttctgagatgccctcttttgttgctgtttcactgttctcacaatatgtggcaagtttgtcaagtgcaattaattctgcattctcaaaaacagaggcctaagtgtcaagagtttccagatgatttcccattcctcaccacttttaggggaaaggcatggtttccaggatttcagctgtgtctttaagggctggaggtggatgtctgttgactcttgggatgctctgagacatgttaaatccttccatggcactgctggtccctgtggactagctgggacctgctgccctgggtcatcaaactccctctctaaatcctccaacagggtcacagcttcctcgccgctttctggattatgttgctgaacccagatctgcagctcctcaggcagaatgctcaggaactgctccagtaccagcagttctaagatctgctcctttgtgtgcaactctggcattagccactgatagcaaagttcctggagtcggctcagagcctcccggggcccaggtgtctcctggtagcaaaattttctgaattgctgacgaaacaattcttggcaggattgagtactcccattctgcttaaatttctcatcccaggaaaagttatcttctactttcactagtattagttcttgttccggaggatcctgaggtatcagggttgaaatcactccagattccacagccattcttggctgaaacagcttagcaaaaagctcagtacaactggttctgtgcttgcgaaggagtgtgagtaatctcttctttccgcgaagcccaggagcggccaggaaatgagccacccaccccgagctgcaagccacaaagaccggaagtgcgcgtac

SEQ ID NO: 15790 - RNA, 5001 nt, Homo sapiens
  source 1..5001: mol_type = other RNA
gctgggattacaggcatgagccactgtgcctggcctgtgacatcagttttaagagtttcaggattttgtgtacattcatgatggttactgaaacatacatttccaggtacaatttcaaagtcaaaaggcaatgcttaaagcttctggtattgattgccagagatggtatgtatttattcatgtcttaccagcagcattagagtcccaatgtccctgaatccctgtctgttttataaggaaaagtgtcatctcaactcttgctttaatatacattttaactgtagtgaggttgaacatttattgttcattggcacttattttgtgatttccctacttaagtagcattttttttctattggaactttcttatggggagagagtatactgaagtggctccacagtcaggttgtgggttcaaagtctgacctccccactttgtagatatatgacctttagccttcatttcctcatctgctacatacgtgctgagaaataacaataataagtatatacaaagcccttagcaagtatctattacatttacttttttcctttttttttggtttggagacagggtcttgctctcccaggctggagtgcagtggtgtgatcttgcctcactgaagcctcgacttccagggctcaagcgaacctctcacctcagcctcccaaatacttgggtctacaggcatgcactaccacgtctggcaaattctgtttattttttgtagagatggggtctcactatgctgcccaggctcggcttgaactcctagactcaagcaatcctccagccttggcctcccaaagtgctggcattataggtgtgagccactgtgcttggtctatctattacattgctttctgacatacagtagagctttcttatataaagagtatttccgttttacaattcctactttacgtcctaccttttcagtttgttcaggtctttatctatggaaaaggagaaaaacaagagttgagtagctcttaccacgtattttaatctcttacatcttttccaaataatcccatccattttttccatattctctccctaaacatgggcatttaggcctcctgctgttcttactggttagcacatgtccactgatgcacgccccaataagagcattacttctctttgcttctttttatcctcatgaaaattctttttctatgcacatgattctagatttccatacagatttgtttttggtgtggtatgttattcttctgacctattaggtcttttgaatatgtctttgtgttgctggttaacctgtacaacattccttcttacactaagcatcagtctaaatattctcttcctgctaggcccctcagaaaagggaagtcttgactgactgtgaccattagtttcagttgtcacttccttttagcattgtctttaataaaatttgcaaaagatggttgggcgccatggctcacgcctgtaatcccagcactttggggggccgaggcgggcggatcacctgagatcgagaattcgagaccagcctgaccaacatggagaaaccctgtctttcctaaaaatacaaaattagccagctgtggtggtgcatgcctgtaatcccagctactcagaaggctgaggcaggagaatcgcttgaacccaggaggcagagtttgcggtgagccaagatcgtgccattgcactccagcctggacaagagcgaactccatctcaaaaaaaaaaaaaaaaaaaaaaaaattgcaaaagatattgtgaaatactggtgacataagacaaaactgaacatgtgcgaggtgcccaaagaatgtcacagacccagcaactgacaaatattttttgagcaccaaagcccaagggaatgtactaggaattgtgggcgtatagccccagaaacaaatgatatggcagcttctgatccagagcgttgggaattttaagaaacctgacagcagctctgatattgtctttagaatcaaaggagaatagagtcttaacactctagcagactcttgaggtataggctgggctctttctcaccctcattcccaccaccaccctcatggaagttctaggatagcctacaggttgggcaaggaaaccacatatttgccctttccctggggtcacataaaccaagacaaagctcttgactaccctgtggcccaagggctccaggttttgtctattaacaggaacttctccattggcactgcttaagagtctggccagacccagacttctctgacagacaagacctcactacaacaggaactcaaggaatgctccacactttgtttctggcctttggctactgttctttactggggtaccacttccctagagtaccaccttggctaactcctcctcatccttcaggccatttcccccatttccttatccaaggctgagtcaggtgctccttaaggtcacataggagcattccactttcactgcctgtctggctgccttgcccattagactgtagagactacagtcttgttttccactgtattcctagttcctgggacaaagtaggtactcaaaaaataacctttgggtaaattatattctttcttctcatgcctatctaattcctggcctgccctgggctcaacaaatcattgatgaagccatttccccacctttcctgctgctctgtcactgttctttattgggtcagttttttttttttttttagttcctgagacgaagtgcctcacacagtccacaccagccccataacctggcacactaacaatcagatgcagtgacagagcctgggttgctatattcatgacactttcatacaaaatgaggtttcaatgttacattcccacttttcgtatttcctgagtattcctaataagagaagagctggaagtaatgattcttctgtattctgttctgattagtcacaggaaaagctttcaagggacactttacattagcactgggaaatgctgcacaaagcaagctagactcaagacctagtattttataacctttatggagttttgctccaaagtaaactcttttgactaacaaacttaaaaatctgactgaagtatttacactattcacagtattcacaaattactttatagtgtggactctttgatggcgcataaggaccgatctgtgcctgaaagccttcccacattcattacatatataagcttcatccccagaatgaattctctgatgctgaacaagggctgagctccttttgaaagttttgccacattcattacactgataaggttcctccccactatgaattctctgatgtctgataaggtttgagctcaaactgaaagcttttccacattcactacattcatagggtttctctccactatgtattctctgatgagtaatcagctctgagctctgcctgaaagcttttccacattcattacattcatagggtctctctcctgtgtgaattcgctgatgtctaatgagttttgagctctggctaaaggttttcccacattcattacactcataaggtttctcaccagtgtgaattctttgatgtataatgagatatgaactttgactgaatgctttgccacactcattacatttacaagctttctcaccagtatggattttccgatgtctaatgagggctgagctctgattgaaagctttcccacattcactacattcatatgctttctcaccactatgaattctctgatgaataataagataggacctcaaactaaaggccttcccacactggttacatttatagggcttttctccagtatggattctctgatgttgtgttagagaggaatgctgcttgaagctgtgcccacatacatcacatctataaggtctctcttctggaggaactttctgacacattatagagtctgtagttagaatcaagcatctttcagcctcatcataaaggtctctctttcctagagatttgtttgtgaagatcacttgactaaaactgcccccttgggaaggagatcttagtttctcccctgtagcacttccttgcttccacactaaattgctttcatgctcactaattcctcgaaatgaaggttcctgagggagtccctgtgatttttcttctgagatgccctcttttgttgctgtttcactgttctcacaatcacttttaggggaaaggcatggtttccaggatttcagctgtgtctttaagggctggaggtggatgtctgttgactcttgggatgctctgagacatgttaaatccttccatggcactgctggtccctgtggactagctgggaccattacatgctccaggctgtaaattccttttcccacatcacttttctccgttcccacctgctgccctgggtcatcaaactccctctctaaatcctccaacagggtcacagcttcctcgccgctttctggattatgttgctgaacccagatctgcagctcctcaggcagaatgctcaggaactgctccagtaccagcagttctaagatctgctcctttgtgtgcaactctggcattagccactgatagcaaagttcctggagtcggctcagagcctcccggggcccaggtgtctcctggtagcaaaattttctgaattgctgacgaaacaattcttggcaggattgagtactcccattctgcttaaatttctcatcccaggaaaagttatcttctactttcactagtattagttcttgttccggaggatcctgaggtatcagggttgaaatcactccagattccacagccattcttggctgaaacagcttagcaaaaagctcagtacaactggttctgtgcttgcgaaggagtgtgagtaatctcttctttccatgtgttcaaaaacatgataggtatcacatacacaaaagcagcaaagagatccgtatcagttctgaaaaagcttagaatatcccaagacgcgaagcccaggagcggccaggaaatgagccacccaccccgagctgcaagccacaaagaccggaagtgcgcgtac

SEQ ID NO: 15791 - RNA, 5203 nt, Homo sapiens
  source 1..5203: mol_type = other RNA
gctgggattacaggcatgagccactgtgcctggcctgtgacatcagttttaagagtttcaggattttgtgtacattcatgatggttactgaaacatacatttccaggtacaatttcaaagtcaaaaggcaatgcttaaagcttctggtattgattgccagagatggtatgtatttattcatgtcttaccagcagcattagagtcccaatgtccctgaatccctgtctgttttataaggaaaagtgtcatctcaactcttgctttaatatacattttaactgtagtgaggttgaacatttattgttcattggcacttattttgtgatttccctacttaagtagcattttttttctattggaactttcttatggggagagagtatactgaagtggctccacagtcaggttgtgggttcaaagtctgacctccccactttgtagatatatgacctttagccttcatttcctcatctgctacatacgtgctgagaaataacaataataagtatatacaaagcccttagcaagtatctattacatttacttttttcctttttttttggtttggagacagggtcttgctctcccaggctggagtgcagtggtgtgatcttgcctcactgaagcctcgacttccagggctcaagcgaacctctcacctcagcctcccaaatacttgggtctacaggcatgcactaccacgtctggcaaattctgtttattttttgtagagatggggtctcactatgctgcccaggctcggcttgaactcctagactcaagcaatcctccagccttggcctcccaaagtgctggcattataggtgtgagccactgtgcttggtctatctattacattgctttctgacatacagtagagctttcttatataaagagtatttccgttttacaattcctactttacgtcctaccttttcagtttgttcaggtctttatctatggaaaaggagaaaaacaagagttgagtagctcttaccacgtattttaatctcttacatcttttccaaataatcccatccattttttccatattctctccctaaacatgggcatttaggcctcctgctgttcttactggttagcacatgtccactgatgcacgccccaataagagcattacttctctttgcttctttttatcctcatgaaaattctttttctatgcacatgattctagatttccatacagatttgtttttggtgtggtatgttattcttctgacctattaggtcttttgaatatgtctttgtgttgctggttaacctgtacaacattccttcttacactaagcatcagtctaaatattctcttcctgctaggcccctcagaaaagggaagtcttgactgactgtgaccattagtttcagttgtcacttccttttagcattgtctttaataaaatttgcaaaagatggttgggcgccatggctcacgcctgtaatcccagcactttggggggccgaggcgggcggatcacctgagatcgagaattcgagaccagcctgaccaacatggagaaaccctgtctttcctaaaaatacaaaattagccagctgtggtggtgcatgcctgtaatcccagctactcagaaggctgaggcaggagaatcgcttgaacccaggaggcagagtttgcggtgagccaagatcgtgccattgcactccagcctggacaagagcgaactccatctcaaaaaaaaaaaaaaaaaaaaaaaaattgcaaaagatattgtgaaatactggtgacataagacaaaactgaacatgtgcgaggtgcccaaagaatgtcacagacccagcaactgacaaatattttttgagcaccaaagcccaagggaatgtactaggaattgtgggcgtatagccccagaaacaaatgatatggcagcttctgatccagagcgttgggaattttaagaaacctgacagcagctctgatattgtctttagaatcaaaggagaatagagtcttaacactctagcagactcttgaggtataggctgggctctttctcaccctcattcccaccaccaccctcatggaagttctaggatagcctacaggttgggcaaggaaaccacatatttgccctttccctggggtcacataaaccaagacaaagctcttgactaccctgtggcccaagggctccaggttttgtctattaacaggaacttctccattggcactgcttaagagtctggccagacccagacttctctgacagacaagacctcactacaacaggaactcaaggaatgctccacactttgtttctggcctttggctactgttctttactggggtaccacttccctagagtaccaccttggctaactcctcctcatccttcaggccatttcccccatttccttatccaaggctgagtcaggtgctccttaaggtcacataggagcattccactttcactgcctgtctggctgccttgcccattagactgtagagactacagtcttgttttccactgtattcctagttcctgggacaaagtaggtactcaaaaaataacctttgggtaaattatattctttcttctcatgcctatctaattcctggcctgccctgggctcaacaaatcattgatgaagccatttccccacctttcctgctgctctgtcactgttctttattgggtcagttttttttttttttttagttcctgagacgaagtgcctcacacagtccacaccagccccataacctggcacactaacaatcagatgcagtgacagagcctgggttgctatattcatgacactttcatacaaaatgaggtttcaatgttacattcccacttttcgtatttcctgagtattcctaataagagaagagctggaagtaatgattcttctgtattctgttctgattagtcacaggaaaagctttcaagggacactttacattagcactgggaaatgctgcacaaagcaagctagactcaagacctagtattttataacctttatggagttttgctccaaagtaaactcttttgactaacaaacttaaaaatctgactgaagtatttacactattcacagtattcacaaattactttatagtgtggactctttgatggcgcataaggaccgatctgtgcctgaaagccttcccacattcattacatatataagcttcatccccagaatgaattctctgatgctgaacaagggctgagctccttttgaaagttttgccacattcattacactgataaggttcctccccactatgaattctctgatgtctgataaggtttgagctcaaactgaaagcttttccacattcactacattcatagggtttctctccactatgtattctctgatgagtaatcagctctgagctctgcctgaaagcttttccacattcattacattcatagggtctctctcctgtgtgaattcgctgatgtctaatgagttttgagctctggctaaaggttttcccacattcattacactcataaggtttctcaccagtgtgaattctttgatgtataatgagatatgaactttgactgaatgctttgccacactcattacatttacaagctttctcaccagtatggattttccgatgtctaatgagggctgagctctgattgaaagctttcccacattcactacattcatatgctttctcaccactatgaattctctgatgaataataagataggacctcaaactaaaggccttcccacactggttacatttatagggcttttctccagtatggattctctgatgttgtgttagagaggaatgctgcttgaagctgtgcccacatacatcacatctataaggtctctcttctggaggaactttctgacacattatagagtctgtagttagaatcaagcatctttcagcctcatcataaaggtctctctttcctagagatttgtttgtgaagatcacttgactaaaactgcccccttgggaaggagatcttagtttctcccctgtagcacttccttgcttccacactaaattgctttcatgctcactaattcctcgaaatgaaggttcctgagggagtccctgtgatttttcttctgagatgccctcttttgttgctgtttcactgttctcacaatcacttttaggggaaaggcatggtttccaggatttcagctgtgtctttaagggctggaggtggatgtctgttgactcttgggatgctctgagacatgttaaatccttccatggcactgctggtccctgtggactagctgggaccattacatgctccaggctgtaaattccttttcccacatcacttttctccgttcccacctgctgccctgggtcatcaaactccctctctaaatcctccaacagggtcacagcttcctcgccgctttctggattatgttgctgaacccagatctgcagctcctcaggcagaatgctcaggaactgctccagtaccagcagttctaagatctgctcctttgtgtgcaactctggcattagccactgatagcaaagttcctggagtcggctcagagcctcccggggcccaggtgtctcctggtagcaaaattttctgaattgctgacgaaacaattcttggcaggattgagtactcccattctgcttaaatttctcatcccaggaaaagttatcttctactttcactagtattagttcttgttccggaggatcctgaggtatcagggttgaaatcactccagattccacagccattcttggctgaaacagcttagcaaaaagctcagtacaactggttctgtgcttgcgaaggagtgtgagtaatctcttctttccccgagctgcaagccacaaagaccggaagtgcgcgtacgcagtgttccgctctcgcgcccttcgggtcctccgccgccccgccccttgctctgaggtagccaatcagagccgcgggctctacagtttccaccgccttctcccggtagccgctagcccggcggaatctccaaggccaggggagggtgcgctaggagtcaggggtccttgtgagcggcggcacctggagggtcccgcatctcgcctgggccgttcccaccctggctttctcctggcaccacccatcattgttggtctcaagtaattcccgaatctcactcccagttttccattaaaatattcagattttcggccgggcgcggtggccga

SEQ ID NO: 15792 - RNA, 4912 nt, Homo sapiens
  source 1..4912: mol_type = other RNA
gctgggattacaggcatgagccactgtgcctggcctgtgacatcagttttaagagtttcaggattttgtgtacattcatgatggttactgaaacatacatttccaggtacaatttcaaagtcaaaaggcaatgcttaaagcttctggtattgattgccagagatggtatgtatttattcatgtcttaccagcagcattagagtcccaatgtccctgaatccctgtctgttttataaggaaaagtgtcatctcaactcttgctttaatatacattttaactgtagtgaggttgaacatttattgttcattggcacttattttgtgatttccctacttaagtagcattttttttctattggaactttcttatggggagagagtatactgaagtggctccacagtcaggttgtgggttcaaagtctgacctccccactttgtagatatatgacctttagccttcatttcctcatctgctacatacgtgctgagaaataacaataataagtatatacaaagcccttagcaagtatctattacatttacttttttcctttttttttggtttggagacagggtcttgctctcccaggctggagtgcagtggtgtgatcttgcctcactgaagcctcgacttccagggctcaagcgaacctctcacctcagcctcccaaatacttgggtctacaggcatgcactaccacgtctggcaaattctgtttattttttgtagagatggggtctcactatgctgcccaggctcggcttgaactcctagactcaagcaatcctccagccttggcctcccaaagtgctggcattataggtgtgagccactgtgcttggtctatctattacattgctttctgacatacagtagagctttcttatataaagagtatttccgttttacaattcctactttacgtcctaccttttcagtttgttcaggtctttatctatggaaaaggagaaaaacaagagttgagtagctcttaccacgtattttaatctcttacatcttttccaaataatcccatccattttttccatattctctccctaaacatgggcatttaggcctcctgctgttcttactggttagcacatgtccactgatgcacgccccaataagagcattacttctctttgcttctttttatcctcatgaaaattctttttctatgcacatgattctagatttccatacagatttgtttttggtgtggtatgttattcttctgacctattaggtcttttgaatatgtctttgtgttgctggttaacctgtacaacattccttcttacactaagcatcagtctaaatattctcttcctgctaggcccctcagaaaagggaagtcttgactgactgtgaccattagtttcagttgtcacttccttttagcattgtctttaataaaatttgcaaaagatggttgggcgccatggctcacgcctgtaatcccagcactttggggggccgaggcgggcggatcacctgagatcgagaattcgagaccagcctgaccaacatggagaaaccctgtctttcctaaaaatacaaaattagccagctgtggtggtgcatgcctgtaatcccagctactcagaaggctgaggcaggagaatcgcttgaacccaggaggcagagtttgcggtgagccaagatcgtgccattgcactccagcctggacaagagcgaactccatctcaaaaaaaaaaaaaaaaaaaaaaaaattgcaaaagatattgtgaaatactggtgacataagacaaaactgaacatgtgcgaggtgcccaaagaatgtcacagacccagcaactgacaaatattttttgagcaccaaagcccaagggaatgtactaggaattgtgggcgtatagccccagaaacaaatgatatggcagcttctgatccagagcgttgggaattttaagaaacctgacagcagctctgatattgtctttagaatcaaaggagaatagagtcttaacactctagcagactcttgaggtataggctgggctctttctcaccctcattcccaccaccaccctcatggaagttctaggatagcctacaggttgggcaaggaaaccacatatttgccctttccctggggtcacataaaccaagacaaagctcttgactaccctgtggcccaagggctccaggttttgtctattaacaggaacttctccattggcactgcttaagagtctggccagacccagacttctctgacagacaagacctcactacaacaggaactcaaggaatgctccacactttgtttctggcctttggctactgttctttactggggtaccacttccctagagtaccaccttggctaactcctcctcatccttcaggccatttcccccatttccttatccaaggctgagtcaggtgctccttaaggtcacataggagcattccactttcactgcctgtctggctgccttgcccattagactgtagagactacagtcttgttttccactgtattcctagttcctgggacaaagtaggtactcaaaaaataacctttgggtaaattatattctttcttctcatgcctatctaattcctggcctgccctgggctcaacaaatcattgatgaagccatttccccacctttcctgctgctctgtcactgttctttattgggtcagttttttttttttttttagttcctgagacgaagtgcctcacacagtccacaccagccccataacctggcacactaacaatcagatgcagtgacagagcctgggttgctatattcatgacactttcatacaaaatgaggtttcaatgttacattcccacttttcgtatttcctgagtattcctaataagagaagagctggaagtaatgattcttctgtattctgttctgattagtcacaggaaaagctttcaagggacactttacattagcactgggaaatgctgcacaaagcaagctagactcaagacctagtattttataacctttatggagttttgctccaaagtaaactcttttgactaacaaacttaaaaatctgactgaagtatttacactattcacagtattcacaaattactttatagtgtggactctttgatggcgcataaggaccgatctgtgcctgaaagccttcccacattcattacatatataagcttcatccccagaatgaattctctgatgctgaacaagggctgagctccttttgaaagttttgccacattcattacactgataaggttcctccccactatgaattctctgatgtctgataaggtttgagctcaaactgaaagcttttccacattcactacattcatagggtttctctccactatgtattctctgatgagtaatcagctctgagctctgcctgaaagcttttccacattcattacattcatagggtctctctcctgtgtgaattcgctgatgtctaatgagttttgagctctggctaaaggttttcccacattcattacactcataaggtttctcaccagtgtgaattctttgatgtataatgagatatgaactttgactgaatgctttgccacactcattacatttacaagctttctcaccagtatggattttccgatgtctaatgagggctgagctctgattgaaagctttcccacattcactacattcatatgctttctcaccactatgaattctctgatgaataataagataggacctcaaactaaaggccttcccacactggttacatttatagggcttttctccagtatggattctctgatgttgtgttagagaggaatgctgcttgaagctgtgcccacatacatcacatctataaggtctctcttctggaggaactttctgacacattatagagtctgtagttagaatcaagcatctttcagcctcatcataaaggtctctctttcctagagatttgtttgtgaagatcacttgactaaaactgcccccttgggaaggagatcttagtttctcccctgtagcacttccttgcttccacactaaattgctttcatgctcactaattcctcgaaatgaaggttcctgagggagtccctgtgatttttcttctgagatgccctcttttgttgctgtttcactgttctcacaatcacttttaggggaaaggcatggtttccaggatttcagctgtgtctttaagggctggaggtggatgtctgttgactcttgggatgctctgagacatgttaaatccttccatggcactgctggtccctgtggactagctgggaccattacatgctccaggctgtaaattccttttcccacatcacttttctccgttcccacctgctgccctgggtcatcaaactccctctctaaatcctccaacagggtcacagcttcctcgccgctttctggattatgttgctgaacccagatctgcagctcctcaggcagaatgctcaggaactgctccagtaccagcagttctaagatctgctcctttgtgtgcaactctggcattagccactgatagcaaagttcctggagtcggctcagagcctcccggggcccaggtgtctcctggtagcaaaattttctgaattgctgacgaaacaattcttggcaggattgagtactcccattctgcttaaatttctcatcccaggaaaagttatcttctactttcactagtattagttcttgttccggaggatcctgaggtatcagggttgaaatcactccagattccacagccattcttggctgaaacagcttagcaaaaagctcagtacaactggttctgtgcttgcgaaggagtgtgagtaatctcttctttccgcgaagcccaggagcggccaggaaatgagccacccaccccgagctgcaagccacaaagaccggaagtgcgcgtac

SEQ ID NO: 15793 - RNA, 4408 nt, Homo sapiens
  source 1..4408: mol_type = other RNA
gctgggattacaggcatgagccactgtgcctggcctgtgacatcagttttaagagtttcaggattttgtgtacattcatgatggttactgaaacatacatttccaggtacaatttcaaagtcaaaaggcaatgcttaaagcttctggtattgattgccagagatggtatgtatttattcatgtcttaccagcagcattagagtcccaatgtccctgaatccctgtctgttttataaggaaaagtgtcatctcaactcttgctttaatatacattttaactgtagtgaggttgaacatttattgttcattggcacttattttgtgatttccctacttaagtagcattttttttctattggaactttcttatggggagagagtatactgaagtggctccacagtcaggttgtgggttcaaagtctgacctccccactttgtagatatatgacctttagccttcatttcctcatctgctacatacgtgctgagaaataacaataataagtatatacaaagcccttagcaagtatctattacatttacttttttcctttttttttggtttggagacagggtcttgctctcccaggctggagtgcagtggtgtgatcttgcctcactgaagcctcgacttccagggctcaagcgaacctctcacctcagcctcccaaatacttgggtctacaggcatgcactaccacgtctggcaaattctgtttattttttgtagagatggggtctcactatgctgcccaggctcggcttgaactcctagactcaagcaatcctccagccttggcctcccaaagtgctggcattataggtgtgagccactgtgcttggtctatctattacattgctttctgacatacagtagagctttcttatataaagagtatttccgttttacaattcctactttacgtcctaccttttcagtttgttcaggtctttatctatggaaaaggagaaaaacaagagttgagtagctcttaccacgtattttaatctcttacatcttttccaaataatcccatccattttttccatattctctccctaaacatgggcatttaggcctcctgctgttcttactggttagcacatgtccactgatgcacgccccaataagagcattacttctctttgcttctttttatcctcatgaaaattctttttctatgcacatgattctagatttccatacagatttgtttttggtgtggtatgttattcttctgacctattaggtcttttgaatatgtctttgtgttgctggttaacctgtacaacattccttcttacactaagcatcagtctaaatattctcttcctgctaggcccctcagaaaagggaagtcttgactgactgtgaccattagtttcagttgtcacttccttttagcattgtctttaataaaatttgcaaaagatggttgggcgccatggctcacgcctgtaatcccagcactttggggggccgaggcgggcggatcacctgagatcgagaattcgagaccagcctgaccaacatggagaaaccctgtctttcctaaaaatacaaaattagccagctgtggtggtgcatgcctgtaatcccagctactcagaaggctgaggcaggagaatcgcttgaacccaggaggcagagtttgcggtgagccaagatcgtgccattgcactccagcctggacaagagcgaactccatctcaaaaaaaaaaaaaaaaaaaaaaaaattgcaaaagatattgtgaaatactggtgacataagacaaaactgaacatgtgcgaggtgcccaaagaatgtcacagacccagcaactgacaaatattttttgagcaccaaagcccaagggaatgtactaggaattgtgggcgtatagccccagaaacaaatgatatggcagcttctgatccagagcgttgggaattttaagaaacctgacagcagctctgatattgtctttagaatcaaaggagaatagagtcttaacactctagcagactcttgaggtataggctgggctctttctcaccctcattcccaccaccaccctcatggaagttctaggatagcctacaggttgggcaaggaaaccacatatttgccctttccctggggtcacataaaccaagacaaagctcttgactaccctgtggcccaagggctccaggttttgtctattaacaggaacttctccattggcactgcttaagagtctggccagacccagacttctctgacagacaagacctcactacaacaggaactcaaggaatgctccacactttgtttctggcctttggctactgttctttactggggtaccacttccctagagtaccaccttggctaactcctcctcatccttcaggccatttcccccatttccttatccaaggctgagtcaggtgctccttaaggtcacataggagcattccactttcactgcctgtctggctgccttgcccattagactgtagagactacagtcttgttttccactgtattcctagttcctgggacaaagtaggtactcaaaaaataacctttgggtaaattatattctttcttctcatgcctatctaattcctggcctgccctgggctcaacaaatcattgatgaagccatttccccacctttcctgctgctctgtcactgttctttattgggtcagttttttttttttttttagttcctgagacgaagtgcctcacacagtccacaccagccccataacctggcacactaacaatcagatgcagtgacagagcctgggttgctatattcatgacactttcatacaaaatgaggtttcaatgttacattcccacttttcgtatttcctgagtattcctaataagagaagagctggaagtaatgattcttctgtattctgttctgattagtcacaggaaaagctttcaagggacactttacattagcactgggaaatgctgcacaaagcaagctagactcaagacctagtattttataacctttatggagttttgctccaaagtaaactcttttgactaacaaacttaaaaatctgactgaagtatttacactattcacagtattcacaaattactttatagtgtggactctttgatggcgcataaggaccgatctgtgcctgaaagccttcccacattcattacatatataagcttcatccccagaatgaattctctgatgctgaacaagggctgagctccttttgaaagttttgccacattcattacactgataaggttcctccccactatgaattctctgatgtctgataaggtttgagctcaaactgaaagcttttccacattcactacattcatagggtttctctccactatgtattctctgatgagtaatcagctctgagctctgcctgaaagcttttccacattcattacattcatagggtctctctcctgtgtgaattcgctgatgtctaatgagttttgagctctggctaaaggttttcccacattcattacactcataaggtttctcaccagtgtgaattctttgatgtataatgagatatgaactttgactgaatgctttgccacactcattacatttacaagctttctcaccagtatggattttccgatgtctaatgagggctgagctctgattgaaagctttcccacattcactacattcatatgctttctcaccactatgaattctctgatgaataataagataggacctcaaactaaaggccttcccacactggttacatttatagggcttttctccagtatggattctctgatgttgtgttagagaggaatgctgcttgaagctgtgcccacatacatcacatctataaggtctctcttctggaggaactttctgacacattatagagtctgtagttagaatcaagcatctttcagcctcatcataaaggtctctctttcctagagatttgtttgtgaagatcacttgactaaaactgcccccttgggaaggagatcttagtttctcccctgtagcacttccttgcttccacactaaattgctttcatgctcactaattcctcgaaatgaaggttcctgagggagtccctgtgatttttcttctgagatgccctcttttgttgctgtttcactgttctcacaatcacttttaggggaaaggcatggtttccaggatttcagctgtgtctttaagggctggaggtggatgtctgttgactcttgggatgctctgagacatgttaaatccttccatggcactgctggtccctgtggactagctgggaccgcgaagcccaggagcggccaggaaatgagccacccaccccgagctgcaagccacaaagaccggaagtgcgcgtacgcagtgttccgctctcgcgcccttcgggtcctccgccgccccgcccc

SEQ ID NO: 15794 - RNA, 4800 nt, Homo sapiens
  source 1..4800: mol_type = other RNA
gctgggattacaggcatgagccactgtgcctggcctgtgacatcagttttaagagtttcaggattttgtgtacattcatgatggttactgaaacatacatttccaggtacaatttcaaagtcaaaaggcaatgcttaaagcttctggtattgattgccagagatggtatgtatttattcatgtcttaccagcagcattagagtcccaatgtccctgaatccctgtctgttttataaggaaaagtgtcatctcaactcttgctttaatatacattttaactgtagtgaggttgaacatttattgttcattggcacttattttgtgatttccctacttaagtagcattttttttctattggaactttcttatggggagagagtatactgaagtggctccacagtcaggttgtgggttcaaagtctgacctccccactttgtagatatatgacctttagccttcatttcctcatctgctacatacgtgctgagaaataacaataataagtatatacaaagcccttagcaagtatctattacatttacttttttcctttttttttggtttggagacagggtcttgctctcccaggctggagtgcagtggtgtgatcttgcctcactgaagcctcgacttccagggctcaagcgaacctctcacctcagcctcccaaatacttgggtctacaggcatgcactaccacgtctggcaaattctgtttattttttgtagagatggggtctcactatgctgcccaggctcggcttgaactcctagactcaagcaatcctccagccttggcctcccaaagtgctggcattataggtgtgagccactgtgcttggtctatctattacattgctttctgacatacagtagagctttcttatataaagagtatttccgttttacaattcctactttacgtcctaccttttcagtttgttcaggtctttatctatggaaaaggagaaaaacaagagttgagtagctcttaccacgtattttaatctcttacatcttttccaaataatcccatccattttttccatattctctccctaaacatgggcatttaggcctcctgctgttcttactggttagcacatgtccactgatgcacgccccaataagagcattacttctctttgcttctttttatcctcatgaaaattctttttctatgcacatgattctagatttccatacagatttgtttttggtgtggtatgttattcttctgacctattaggtcttttgaatatgtctttgtgttgctggttaacctgtacaacattccttcttacactaagcatcagtctaaatattctcttcctgctaggcccctcagaaaagggaagtcttgactgactgtgaccattagtttcagttgtcacttccttttagcattgtctttaataaaatttgcaaaagatggttgggcgccatggctcacgcctgtaatcccagcactttggggggccgaggcgggcggatcacctgagatcgagaattcgagaccagcctgaccaacatggagaaaccctgtctttcctaaaaatacaaaattagccagctgtggtggtgcatgcctgtaatcccagctactcagaaggctgaggcaggagaatcgcttgaacccaggaggcagagtttgcggtgagccaagatcgtgccattgcactccagcctggacaagagcgaactccatctcaaaaaaaaaaaaaaaaaaaaaaaaattgcaaaagatattgtgaaatactggtgacataagacaaaactgaacatgtgcgaggtgcccaaagaatgtcacagacccagcaactgacaaatattttttgagcaccaaagcccaagggaatgtactaggaattgtgggcgtatagccccagaaacaaatgatatggcagcttctgatccagagcgttgggaattttaagaaacctgacagcagctctgatattgtctttagaatcaaaggagaatagagtcttaacactctagcagactcttgaggtataggctgggctctttctcaccctcattcccaccaccaccctcatggaagttctaggatagcctacaggttgggcaaggaaaccacatatttgccctttccctggggtcacataaaccaagacaaagctcttgactaccctgtggcccaagggctccaggttttgtctattaacaggaacttctccattggcactgcttaagagtctggccagacccagacttctctgacagacaagacctcactacaacaggaactcaaggaatgctccacactttgtttctggcctttggctactgttctttactggggtaccacttccctagagtaccaccttggctaactcctcctcatccttcaggccatttcccccatttccttatccaaggctgagtcaggtgctccttaaggtcacataggagcattccactttcactgcctgtctggctgccttgcccattagactgtagagactacagtcttgttttccactgtattcctagttcctgggacaaagtaggtactcaaaaaataacctttgggtaaattatattctttcttctcatgcctatctaattcctggcctgccctgggctcaacaaatcattgatgaagccatttccccacctttcctgctgctctgtcactgttctttattgggtcagttttttttttttttttagttcctgagacgaagtgcctcacacagtccacaccagccccataacctggcacactaacaatcagatgcagtgacagagcctgggttgctatattcatgacactttcatacaaaatgaggtttcaatgttacattcccacttttcgtatttcctgagtattcctaataagagaagagctggaagtaatgattcttctgtattctgttctgattagtcacaggaaaagctttcaagggacactttacattagcactgggaaatgctgcacaaagcaagctagactcaagacctagtattttataacctttatggagttttgctccaaagtaaactcttttgactaacaaacttaaaaatctgactgaagtatttacactattcacagtattcacaaattactttatagtgtggactctttgatggcgcataaggaccgatctgtgcctgaaagccttcccacattcattacatatataagcttcatccccagaatgaattctctgatgctgaacaagggctgagctccttttgaaagttttgccacattcattacactgataaggttcctccccactatgaattctctgatgtctgataaggtttgagctcaaactgaaagcttttccacattcactacattcatagggtttctctccactatgtattctctgatgagtaatcagctctgagctctgcctgaaagcttttccacattcattacattcatagggtctctctcctgtgtgaattcgctgatgtctaatgagttttgagctctggctaaaggttttcccacattcattacactcataaggtttctcaccagtgtgaattctttgatgtataatgagatatgaactttgactgaatgctttgccacactcattacatttacaagctttctcaccagtatggattttccgatgtctaatgagggctgagctctgattgaaagctttcccacattcactacattcatatgctttctcaccactatgaattctctgatgaataataagataggacctcaaactaaaggccttcccacactggttacatttatagggcttttctccagtatggattctctgatgttgtgttagagaggaatgctgcttgaagctgtgcccacatacatcacatctataaggtctctcttctggaggaactttctgacacattatagagtctgtagttagaatcaagcatctttcagcctcatcataaaggtctctctttcctagagatttgtttgtgaagatcacttgactaaaactgcccccttgggaaggagatcttagtttctcccctgtagcacttccttgcttccacactaaattgctttcatgctcactaattcctcgaaatgaaggttcctgagggagtccctgtgatttttcttctgagatgccctcttttgttgctgtttcactgttctcacaatcacttttaggggaaaggcatggtttccaggatttcagctgtgtctttaagggctggaggtggatgtctgttgactcttgggatgctctgagacatgttaaatccttccatggcactgctggtccctgtggactagctgggacctgctgccctgggtcatcaaactccctctctaaatcctccaacagggtcacagcttcctcgccgctttctggattatgttgctgaacccagatctgcagctcctcaggcagaatgctcaggaactgctccagtaccagcagttctaagatctgctcctttgtgtgcaactctggcattagccactgatagcaaagttcctggagtcggctcagagcctcccggggcccaggtgtctcctggtagcaaaattttctgaattgctgacgaaacaattcttggcaggattgagtactcccattctgcttaaatttctcatcccaggaaaagttatcttctactttcactagtattagttcttgttccggaggatcctgaggtatcagggttgaaatcactccagattccacagccattcttggctgaaacagcttagcaaaaagctcagtacaactggttctgtgcttgcgaaggagtgtgagtaatctcttctttccccgagctgcaagccacaaag

SEQ ID NO: 15795 - RNA, 4855 nt, Homo sapiens
  source 1..4855: mol_type = other RNA
gctgggattacaggcatgagccactgtgcctggcctgtgacatcagttttaagagtttcaggattttgtgtacattcatgatggttactgaaacatacatttccaggtacaatttcaaagtcaaaaggcaatgcttaaagcttctggtattgattgccagagatggtatgtatttattcatgtcttaccagcagcattagagtcccaatgtccctgaatccctgtctgttttataaggaaaagtgtcatctcaactcttgctttaatatacattttaactgtagtgaggttgaacatttattgttcattggcacttattttgtgatttccctacttaagtagcattttttttctattggaactttcttatggggagagagtatactgaagtggctccacagtcaggttgtgggttcaaagtctgacctccccactttgtagatatatgacctttagccttcatttcctcatctgctacatacgtgctgagaaataacaataataagtatatacaaagcccttagcaagtatctattacatttacttttttcctttttttttggtttggagacagggtcttgctctcccaggctggagtgcagtggtgtgatcttgcctcactgaagcctcgacttccagggctcaagcgaacctctcacctcagcctcccaaatacttgggtctacaggcatgcactaccacgtctggcaaattctgtttattttttgtagagatggggtctcactatgctgcccaggctcggcttgaactcctagactcaagcaatcctccagccttggcctcccaaagtgctggcattataggtgtgagccactgtgcttggtctatctattacattgctttctgacatacagtagagctttcttatataaagagtatttccgttttacaattcctactttacgtcctaccttttcagtttgttcaggtctttatctatggaaaaggagaaaaacaagagttgagtagctcttaccacgtattttaatctcttacatcttttccaaataatcccatccattttttccatattctctccctaaacatgggcatttaggcctcctgctgttcttactggttagcacatgtccactgatgcacgccccaataagagcattacttctctttgcttctttttatcctcatgaaaattctttttctatgcacatgattctagatttccatacagatttgtttttggtgtggtatgttattcttctgacctattaggtcttttgaatatgtctttgtgttgctggttaacctgtacaacattccttcttacactaagcatcagtctaaatattctcttcctgctaggcccctcagaaaagggaagtcttgactgactgtgaccattagtttcagttgtcacttccttttagcattgtctttaataaaatttgcaaaagatggttgggcgccatggctcacgcctgtaatcccagcactttggggggccgaggcgggcggatcacctgagatcgagaattcgagaccagcctgaccaacatggagaaaccctgtctttcctaaaaatacaaaattagccagctgtggtggtgcatgcctgtaatcccagctactcagaaggctgaggcaggagaatcgcttgaacccaggaggcagagtttgcggtgagccaagatcgtgccattgcactccagcctggacaagagcgaactccatctcaaaaaaaaaaaaaaaaaaaaaaaaattgcaaaagatattgtgaaatactggtgacataagacaaaactgaacatgtgcgaggtgcccaaagaatgtcacagacccagcaactgacaaatattttttgagcaccaaagcccaagggaatgtactaggaattgtgggcgtatagccccagaaacaaatgatatggcagcttctgatccagagcgttgggaattttaagaaacctgacagcagctctgatattgtctttagaatcaaaggagaatagagtcttaacactctagcagactcttgaggtataggctgggctctttctcaccctcattcccaccaccaccctcatggaagttctaggatagcctacaggttgggcaaggaaaccacatatttgccctttccctggggtcacataaaccaagacaaagctcttgactaccctgtggcccaagggctccaggttttgtctattaacaggaacttctccattggcactgcttaagagtctggccagacccagacttctctgacagacaagacctcactacaacaggaactcaaggaatgctccacactttgtttctggcctttggctactgttctttactggggtaccacttccctagagtaccaccttggctaactcctcctcatccttcaggccatttcccccatttccttatccaaggctgagtcaggtgctccttaaggtcacataggagcattccactttcactgcctgtctggctgccttgcccattagactgtagagactacagtcttgttttccactgtattcctagttcctgggacaaagtaggtactcaaaaaataacctttgggtaaattatattctttcttctcatgcctatctaattcctggcctgccctgggctcaacaaatcattgatgaagccatttccccacctttcctgctgctctgtcactgttctttattgggtcagttttttttttttttttagttcctgagacgaagtgcctcacacagtccacaccagccccataacctggcacactaacaatcagatgcagtgacagagcctgggttgctatattcatgacactttcatacaaaatgaggtttcaatgttacattcccacttttcgtatttcctgagtattcctaataagagaagagctggaagtaatgattcttctgtattctgttctgattagtcacaggaaaagctttcaagggacactttacattagcactgggaaatgctgcacaaagcaagctagactcaagacctagtattttataacctttatggagttttgctccaaagtaaactcttttgactaacaaacttaaaaatctgactgaagtatttacactattcacagtattcacaaattactttatagtgtggactctttgatggcgcataaggaccgatctgtgcctgaaagccttcccacattcattacatatataagcttcatccccagaatgaattctctgatgctgaacaagggctgagctccttttgaaagttttgccacattcattacactgataaggttcctccccactatgaattctctgatgtctgataaggtttgagctcaaactgaaagcttttccacattcactacattcatagggtttctctccactatgtattctctgatgagtaatcagctctgagctctgcctgaaagcttttccacattcattacattcatagggtctctctcctgtgtgaattcgctgatgtctaatgagttttgagctctggctaaaggttttcccacattcattacactcataaggtttctcaccagtgtgaattctttgatgtataatgagatatgaactttgactgaatgctttgccacactcattacatttacaagctttctcaccagtatggattttccgatgtctaatgagggctgagctctgattgaaagctttcccacattcactacattcatatgctttctcaccactatgaattctctgatgaataataagataggacctcaaactaaaggccttcccacactggttacatttatagggcttttctccagtatggattctctgatgttgtgttagagaggaatgctgcttgaagctgtgcccacatacatcacatctataaggtctctcttctggaggaactttctgacacattatagagtctgtagttagaatcaagcatctttcagcctcatcataaaggtctctctttcctagagatttgtttgtgaagatcacttgactaaaactgcccccttgggaaggagatcttagtttctcccctgtagcacttccttgcttccacactaaattgctttcatgctcactaattcctcgaaatgaaggttcctgagggagtccctgtgatttttcttctgagatgccctcttttgttgctgtttcactgttctcacaatcacttttaggggaaaggcatggtttccaggatttcagctgtgtctttaagggctggaggtggatgtctgttgactcttgggatgctctgagacatgttaaatccttccatggcactgctggtccctgtggactagctgggacctgctgccctgggtcatcaaactccctctctaaatcctccaacagggtcacagcttcctcgccgctttctggattatgttgctgaacccagatctgcagctcctcaggcagaatgctcaggaactgctccagtaccagcagttctaagatctgctcctttgtgtgcaactctggcattagccactgatagcaaagttcctggagtcggctcagagcctcccggggcccaggtgtctcctggtagcaaaattttctgaattgctgacgaaacaattcttggcaggattgagtactcccattctgcttaaatttctcatcccaggaaaagttatcttctactttcactagtattagttcttgttccggaggatcctgaggtatcagggttgaaatcactccagattccacagccattcttggctgaaacagcttagcaaaaagctcagtacaactggttctgtgcttgcgaaggagtgtgagtaatctcttctttccgcgaagcccaggagcggccaggaaatgagccacccaccccgagctgcaagccacaaagaccggaagtgcgcgtac

SEQ ID NO: 15796 - RNA, 5836 nt, Homo sapiens
  source 1..5836: mol_type = other RNA
gctgggattacaggcatgagccactgtgcctggccttttctattacctttaaaagttacttcacatagtaaagaaattaggactgattcttggcataaaggagggtacaaaaaaaaattgtgccaggtacagtggctaatggccataatcccaacactttgggaggcggaagtgggcagatcacttgagcccaggagttccagaccatcctgggcaacatggtgaaactcgtctctattaaaaatacaaaaattagccaggcgtagccagtcatacacgcctgtggtcccggctactcgggaggctgaggtgggaggatcacttgagcccagtaggtggaggctgcagtgagctgagatcgcgccactgcactccagcctgggcaacagagtgaggccctgtctcaaaaaaaaaaagaaaagaaaagaaaatttggtttcctggcagatagagttttaacaagcgcatcaagcagtaataatttgtggtcttgtgctcaattctcacacatgatctttgcaagcgtcccagcagccatcacagctctactttcacatgcatgggacacagcacagagcagcagccttgaaaggactgcaaagaggtgtgaattccaaacattctcttaagtcctaacatttctgttcttcattttgtgtgacagaagcccatggaaacaaggcgatgacggcgcttgagggtgaccagacctcctcaatcattccatcagccacccaggactcaacagcagaacctcagaggactcagctgaaagaggttttcactcgagcactaaccacagagaaatgggaagtgccatcctgctgtcatacgcagccgatggctgggtaggactaaatgcccttctgtggtgagatgaaccaagacggcagatgggggaataacatcagtgagagagagattacgaatggatccttgtattgcagatcaaactgggttgtctcttctcaaaccacccaggcagtttctgaatgtcccaagataggggtaggagaaaagaaaaaaaagacaaaacaggagacggtgggtaagaaaacctaaaaggcacaatgaggcaaaggcctaagatggaggctggctttgggatctgaaatccggccacaatcctccttgttttacctcaagtccaagaattgtcaaaaagaaaacccagaagggctattcattctaaattttaaaatcttttcttcctggcctaccaagtccttgtgttttctttctaggcgcccataaatacaaccccattacagttctatttggctaataatttacagaacatttaaaataccgggtaggtgaacatctcttcatggcttttgtgtaagggcctgaagcgaagagaaaaacaactgattggagattcctatctggcgccttctccagggaaactgacaaccagagaaatctgttgctaggatttctaggacatctggaaattccctttttgttctttctcaacaatataaaatggtatattcgcaaacctatctgaatcacctcaatctaggccactttgaaaatttcatttaaaaatgtaatcacagatttttaaactaattacccaatttgcaaacaaatcccagctacttctggtcttgaacatggagcaaaggtgtgtcagtaaggccaacattcttaggttgacagagacaggttaacacattggctggcttcatttacccccctgccacgccccacactgagctggatgatttgatgggaagagagggtccccacctcagggttcacttccccagccccagcgttcatgggttttcaggaggctcagcctgtgaaaaagaaccaatgatgatgcacaccctggctgaagtgacatctggccaaaggattccaacagaatgaattccatcaacatggaaaagataatccatggcaccaattctgtgctgcttacaggcaatggttaccaaatgagtcaaaacatggcctagaagtggagccgggcccaatgaaaagcctgagttcacacgtgctaggggctccactgaccggcctctgcagcccagcacccagtcctcttgctctgggtgcaaggtgaggaggcagagtgcacacaccggctcctgtgtccccggcctggctggcaatggtaaaatgggctgcctttcttttgcagcttcttctaatcgaaataccaaagggtactgacctctggcctcagggatgtgacttgcagtgcaaattttacctcttcagtgcagagagtggtcttgaaatcttgccagtgtgtggccctccctcagctcctgccaccctggggagccaggatgctgaaatgcataaggcaaaagcactgaatcggatctattccccactgacctttagttacgatcactctgccctgaccagctggagttgggcctgtgtgaagccagtgatttccaacacactgaagaaggtatctgagtccagtgtgaaagccaaattcctcctgaatctgtgatttggtgaagctctgtgaggtattttttgtgtgtggaagactgaaagtgaagggaaacaactaaaaaaattaaacagacaaaagcagtgtaccttatcctggtttcttcaaacataatgcctgtgccaagaattgggcaggagagaaaccaacgaaatgaatataataacttatcctgaggcgctccctcccacgctggcttagagatctcgcacacacaaaaactctccttgtttataagaagctgtctctcagtatgcgggcagctcttcccaaaagcccgtcattaaataagctaaaaacaggtgcaagcgatgtacctgcatgggttcctgagacttgccttgcagaagcggccttccaagtcaccaactcttgagaactccagagaaaaacagcgcaaacacgtgggcaaaaaaaaaaatcctggtgcctgcaccaagttcttctcccaaagtatgttttactcacatagggcaaatttctgtcgcggactcagctgcctttaggagagtaaggatttgaaggggtacagagaatgctgtcagtgtctaaggaggaaaccctgcctcacctatttcaaatcttgactctggttttctaagcaaatttatcttaggatacaaagcacacattagagcttccttcttgccttaatgcaattaaatttgcagccattctgcagaagaactgaagctctcaggtgaaaagaagccttaaatcatgccatgatatatgtcgggggagggaacatttgggtataggtattttcctgaaggaagagaaagggttgaatgtattggcagctgagctgtcccttcaaggggatattgtgaaacaagctcaataaaaacctctccctctgaagcatgaaatgttcccagaggggacaggaggattcctttggtgctatgatgcaacctcaggtcatgtgctcgcacatgctggagcattttcctgagtaacctgaggaaaatgtggcaacagagaaaagcacttggaaaatacacgcaggaggcaggtagtgttcacctccctggttaaaggaaaggcaccccccacatgctcacaggaactctccctcctgcccctcctcttcccctaccccacttccaccccaggggccaccggaagcagcagcagcaaccccggctcctcatcccctgccgtgatgtctgcaagtggctctggctagaagtggtgctggtgaagggctgtagatgagggtctcttctccagcctcttcacgtggcaggagtgacagaacaggtggtcctccagcggataacagcggtggccatcttcatcattgagctccagaccacagtcctcgcagtggtaacactccacgtggtagtctctgtccatggacacgacacggatggtctcatctgagccctcaggtggaaggatgggaagcccacaggctgcacacttgggggccagcaccttgtggtaatctcggacacagtagatcttgttctctgagtccacggtgaagggcaccccatccaaacactcattacagatgacacagcggaaacagccggggtggtaggacttccccagggcttgcaggatcatgtccatgatcagatgtccacaaagaaaacacctgtcagccgactgctggaaaccagagtacaggaagtcttcttcacaaaacactttgccgttgacaaaataaaaggcttttcctctcagcttccggctgcaagctgcacaggtgaagcatgtgtcatggtagaggttccccatggcctgacaggcctggccagccccaaacacccctttgctgcatttcacacaggctccaaagtaatcagccttcgggtgagcatccatctctcgctccagacgttgggtgagggcttctaatttcaactcagcagcagagggtctcagctcaggacctgggacgaggggctggcagggcagccttaccctaggggagctggggctgtccaggagcacagatcccaggctaccatcagaagaccagcccaggggaccctctttacaagataactcaggcagggtggacatcactggatggacaagactggtggggctgagcttgggaccagtgccaaggtctgtgcagccaggcttcggccccagcccagggaccgcaccctgctgtgaaccgtccagaccagctggcgaggatgacggggcagaactggaaaggtaagatttgggcccatcctggaaccagggttgggggtccacattgggtttggacatcacacctgaaacctcaccccccagccccgagtttgatcttggaagacctccttgcctggggcagctcagggccaagggtgctgacacagaaggggtcctgggctgaacaggccccacagctggtgctccgttctccaagtttggggaaggcaggccagggctcacccgctgggaggaggcagtggaccaaaggcctgttggcttctcgctgctgcggccaccaatgccactattctgaccaccgaggctaccctcagaagacctgctggagctcagggagagctgtcggtgatttaggggatggtccccgcagggtttgggcagtggtgggtcactccccggggagctaggccacccactccctacactcaggccgatgctgggggacactcctggtttgtcaccccactttgggcttgccaaggagaggttgtcataatagtctccatgagtgaggcaggaaggatcctcacaggggcctggctggtggaaagcagacatctcagaagtcgccaggctctccctggaaccacagtcctggctgccatgcctcgtgccatgcaggtatggcctggatctctgctcctgcggtgggtacgggggctgcccagcagcgagggtggtgactgccccaggtgcccctgtcgaggcagcaagaggaggcttggcagcaccatccacagtcagcttgctgcccacaacttcccaacgggcctgtgggcccaggcggccccctccattgacagggcctctactccccctgggcagagtctcctcctgcaggagctgctgctgctgctgctggaggtggattttggccatcttggtggcgaacaccctgcgagtttcctcaaactcggggttgttgcctgcacccttgtccactcggaagagcccatccttagaggcctcatacatgttcaggtcctcgatgaatttactggcctccaggcccaggtcgtcatacttatccatgctgcagacaggtgtccgggcctagcccaggtgccgtgtgtgtgtgtgtgtgtgtgtgtgtgtgtgtgtgtgtgtgtgtgtgtgtgtgtgtgtgtgtgtgttgagggcagcggggagatgctggcgaag

SEQ ID NO: 15797 - RNA, 1401 nt, Homo sapiens
  source 1..1401: mol_type = other RNA
gctgggattacaggcatgagccactgtgcctggctacctgtgcgaataaacttctaacagctctacattgcctttcaaaatctgactcaatttaccttactacttccaaatcgtgcaacttctctgcttaactgtaagctccttcagggcacagaccatgccttttcttctgtgtatccttaatttcttttttttttatttctttctttctttcttttttttttttttgagacagagtctcactgtcgcccaggctggagtgcaatggtgcaatctcggctcatggtagccttcttctcctgggttccagcggttcttctgcttaagcctccagggtagctgggattacaggcatgcgccactacacttggctaatgtttgtatttttagtagagacggggtttcaccatgttggccaggctggtctcgaactcctgacctcaggtgattcacctgcctcagcctcccgaagtgctgggattacaggcatgagccaccacacccagccccttaatttcttatatagtgcctagcacacagaagatgctctataaatagttactgaatggacaaatgactaaactttgaaacttctttgaccttactatgctcaaatatcacttctgatgttcttctccgactctctcacttatcttatatatgtctgcacacgttttttcctcattagactgtaaggtccattctgagcaggatctgttctacccagaccacaggtttctgcctttttttctggctcatcaagcaggcatgtttacccactctttttatcttcatgtttcccaggtcagcccaatgtgaggactttaagtagtagaaggaagtttcgatggtgacggacagtcactttctagagctcagatcactgctgcctccagcacttgtgggatggaaaaaatgaagaaattacagttgccctaaaaatgtcccccacttcaggaacctgaatattttacacagcaggagatacatcggaagtcctacagaatctcttgactttgggagatgcaactgcttttctattaggataacctaattttctgtgtccattttctcagaatgttgtgcccaacgcgttctgtttcctaaatacccagccttccttctggtagaggcaagaaaattatgctagcattcgctcactgcatgttttgagcgtttgagttcagagtacagctattctctctcctcgtaatgtaaacacaggttcccacggcggcaatgggagactcccctaaggggctcttgacgtacagggagacttccagatatggtacacagatgtcacattgctagaacgtctctagacggcaacgaaacattaaagcctaacctgaggtaatccctcaccggcagtgaagctcctctgctaggcactgtcgt

SEQ ID NO: 15798 - RNA, 4083 nt, Homo sapiens
  source 1..4083: mol_type = other RNA
gctgggattacaggcatgagccactgtgcctggctccactttatcttcaatgtctctatttcctcttgtttaaatacaatggctaataagtctagaataacgctaagtaataacaccacactatggtcatgagttcaggttgggctatttataatataatcaatacctatgatgaaaccactgtccaacctcaaactagataattgctgataacaatacagacttattttacttgccatcctcttctcaccaccaaagtaaacattattgggaatttttatcattcttttgttttttatcatatatataatatacacacacataatagtcaattctcattttttgcagactccgtatgtgtgaatttacctcttgctaaaatttatttctaactccagtatcagtacttgctgggcttttgcagccatttgcggacatgcagcatgtgaaaaaatttgaattgcctgctctccatgttcccagctgaggtggaacaaggccttcttgtttcagttcttataaacaagtatccttttcagtctatttagtgccatgtcttttgcatttttgtggattttgctgcttaaagtgacccccacgcacagtgccaagtgttcctaagtgcaagaagactgtgatgtgccgcctggagaaactgaggtaagcttcattcaggaataagtgtcgtgggctaagttcagtgttaatgggtcaaccatatatactaaggtgtcttcaaacagaaacacatgtaacaagtttatgtactgatgggttgatgaaactgtgcccagaggttcataggaacccaaccctgtatttcccttgggaataatggttcagtactctctaattcagtgttcatggtgactttataaaacataactactatagataatgagaacagactatacatatatatatacacacacagtcaccgtttagtatccgtggaggattggttccagaaccttccttggatataaaaatcctctgatgctcaagtccctaatatgaagtatttggatataacctgtgcataccttctcatatacttttaagtcatctctagattacttataataccgaatacagtataaacaccatctaatactttgtattgtttagggaaaaatgacaaggaaaaatgtctgtacaggtttagtccagacacaattttccccctcaatattttcaacctgtagttggttgagtccatagatgtggaacccacatatacagacagccaaccgcatgtctaaacaagtttcacttgtttttgaacttctggagtatcataatgtacatgtcttctgacaccagcttttttcattcaacattattattaacattcacctatattgttactcacagctgcaggacaactttatgtccttgttttagatgtgtctcctgtaaacagcatatgattggggtttgttttaatattcaatttttccttgggctagtttaatacttatacatttattgtaattactgatctatttggacttgttttgccatcttttgttttatccaccttttctatgcttatttctcaaatttaaaattttgtttcttccctattatcccaccatctctcatcactattcattgagagattatatatacttctagcaattaacctcggaattttatcatgcatacttaaaaagactaagttgatattaactggctactcccaaaaatgtaagaacactgaaacattttgactctgattaaccttcccaccatgctgtctacttttaacctacctttaacaatttggcctgtcattatcattttgccgataagatctgtttacatttccctacctgtaagaaattatctatcattactatccacactttatgactcccataacttatatttcctgaggtacatatctcagaactgagttccaggctggggttcatgttgcttattactttcaaactattcacctttaggcatcatagtatctaccacttatctgtgcttactacataccaggtgatattctccacaagtgttgattaacctgacatttattaattcatggaatcctcataataccctaatggactatgtatgtttatgatccatatcttatgactcttataatttatctttcctaaggctacacatacctcagaactaggatccaggcctttttgattccccattgccttcactcaccttttcactccaacgtataatttcctgagttcttgaataatgacttatttctaagacacacagtggcgaggcggaactccaggataccagaggaaatggatgtctgaagttacacaggcaagtactctagcctacaaggcctctgggaaatgccatctagtctttgcttaaattgagccactggcagacctcagtataactcaaggctctatcctcgagttacagatagcacctaagaattttctgaagttttggggaaacctctttaatctttaacccacagatcttaattctgcctccccgaaccaaagtggcaaagagctccatcttactattaatgtattttaagatagtgactacacactctactcttttagttcagattaagcatccaattttcttagctattttttctccatggattcttattttcatttcctgtagaaatcacatgaatcctcaagaaaaggttgttttgccaatggacacctttccatattgaaaaccaaaagaacagtttggtaaaacagtaacatgccaaacacataaccaacttctctacctacaatattcacttcctagtttctgtgtgatctaaaacattttcctcccttccacccggcaataaactcacataagatgaaattaatttacaaaaggtaggctccgtttattagagtcacacacaactgactatctcagtgtgactcaagaccacaaaaaacccatttctccttcacttctgagtcctggggttaatacctagaccagcaagtgtactgcttggggtccattcacaggtttacaagtttttcattgagtgcaatctgtgactgtgtgaggttggccaggtaggtcaccatcaaaaggtcattgatgttgctgttgagcatggtctcaaagtcatcgggaactattttcggtacttggttaaccaggctcatcaggaagcggcccacagtattgtcagctgacacctttccagacagtacatcctctgcatattgcaacactgtactcagggcatcctggatgcgagctgatgcccctcctacttgctgcaagtcacttgagagtccaatcactctgttggggctaaagcaggtcttcatgatcaggtcaactccgatgcgttcagtgtcgtagtacgcgtatttcactgtcagaggcgtgaacatcactcccatggtcctcccagggactcccattaaagtgctgacgtaggctttgatgctcatgcggccgttctggagacttgtgtccacagtgaggtggatggggttgggggcctctcggctgtagtactcgtggatcagcacagagtgctctgtgatgtcatggcccgtagcgtaccagcccaggatgagctcatttggagaaacttttttatgcagttcatacatattcttagcaaattccatgtcaacagccacttcatcttctgactcattgtgcggcactgaaaagcaattggtgacctccactgagtgtttgtcgacagttcccaacagggtcccgataactcgggcagcaccctcgttgcgtctctcgtagctgtccacaatggaggccaaaatgactgggtgcagcctgaccacgcggccgccggggaagggccctggaagagcaggaccaggcagagcgggcgctggggtctgcgctggagcttgcgctgaggccggggtctggccaggagccgcagttgcagccgctgctgccgcagggtctgaggatgaggctggagccgcagcgggaaccggagccgcagccggtgctggcgttggcgctggaactgaggctggggccgccgccgggactggggttggcgtggccggaggagcacttactggtaccgccggtgtggccatcttgtcgagaaagaag

SEQ ID NO: 15799 - RNA, 1387 nt, Homo sapiens
  source 1..1387: mol_type = other RNA
gctgggattacaggcatgagccactgtgcctggctcgctcttcctctcttgaagcaaccaatgttattcgttttatgtggaccatcccagggctatcattattaattcaggtgtttatacaaggctctctgagaactcagttttaaagattacccaaagagtccctgcaacaatccagcctaaaacgatataaaatcagttttaatataactgaagtttttagattctgcctccaaatatcagattgtgacattttacctttctctgactttatgccaaatttacttcaacttctagcatctatcgttctcatttaggaacaaatatgtatttcacaaatgtggaaatacaaccatgagccaaacaaaaccaaatcctggacttacggagctgatggtagattccccaacataaccacttgattacagttttatgcaatgtgatgggagtaagggaccaccgtagggaggtcagaagttgcctctcagaggtggagactacagctgtcgtcagaaggatgagggttggaagaatcttcaggcacagagcaaagcatgagcaaaagctctgtggagtccaggaagctgagtaaatagggaataaaagaggccagtttggctgaagcagagagagcaggatggaattggtctgacctgtaagaagacatggagaggtgggcaaagcgcctggccattcagggcttggttagttaggaggttttgtctaagagaacgggaaggtgtttaagtggtttgggctgggaagtgacagggtcacattacattttgaaaaagccactctgcctgttgtgttgagattagagaggcgataaaggggatatgggtaaaccacaaggagactaggtcagtagtccctccacccccactccccaggtgaaggtagcctagactagggtggtgatggaggaggtagaagaggacagattcaaggaaaatttggaaggtaaaaaccagtaggatttgctgatggacggaatataggaggggaaaggtagattatcagggatgtatcttagttttcttatagaagatgtatttagttgcaatgcaattgttaattgaaattgactttaaataatggcacgacttaaaattatgcaaacatttgccttagataaaatttcaagttttcaaagtttttagctgggtagatggcatggctttacttcatatttcttggtatttcctaatcttgttaaaaaaaaagtttttctttttctcaaaggcttatttcagtggaagcccatctgcgaaatctgttataaatttaaattagaaaataaatacaagtgccattgacacgttggttattgtttttgcgagtgacctaaggccacctctcgcgggagctgggggctgccttccga

SEQ ID NO: 15800 - RNA, 2526 nt, Homo sapiens
  source 1..2526: mol_type = other RNA
gctgggattacaggcatgagccactgtgcctggctgcttctcatttctcaaccccatggccaacctcccccaactccaactcactgctcttgcccaccattttcttttgctgacttctatccatccttcaggtttctgcttataagttaccttctcagggaagtctttcctgattacccagtctaagtctagttttttcaaatatgtatatttaagattgatgtattgttaacatagttcttcccctctatacttaaagctccatgaagaaaagactaatgtttatatttatttgctctctgattcatttctagcagcatctggcagagtgaatatttaataaatatttggtgaaaagatggatgaataaattctaggttaatatttttaattcctttaaagagtttctttgaagagcactttttttccctccctaaattccaatcaacaaattttaaagagagtgtttttaagtaatgttagtgatggtcttgcatcattccgaaagtttaaaaaaaatgtaaaatagaaagaaaagaaaagaaacaacaaacaccattgtacctgaattctgtggaggttaacatgggtcattctgatagacagtcttgttccctaaatctctgatgaatttgcaagaccagatcatagctcaaaaatggattgactacattttctttttctccctctttatagataatatataggtaggttttcatatgttaaattcatgggtgactctgttataatctaatgaaaatgttgcttaatttcaattaaatttattgagcatgtttctatatcagttttatgcaagatgctgtaccaagcataggaaatttcttcacagaatataaactccaaggtggcgagaccatatctactctgctcaacattgtattctccaaggcagaacactgacactgacaaagtaggccttaatagatacttgtgattgaatatatgcacaaatggattacaaagatttacaaggcatattctctggtctttaagaaacttatgatataatagtaggataagctaaatttcaggtctcagacctgagatcaaacattcaagaaagaaaagtatcagagacgtcaactaatatgtgagaaattgcacaactttaccaaccatttttttttaccagccgcattttacaaacatattctctggtaggaaacagttggagagcagtcccaatccagagcaattctcagtgtcttaaacccaagagacatctagcaaagcagtgttttctgattcttgtgcctgaagggtctctctttatctgttcacatttcatggatgttcaataactgagtaatgtacatggagtgttttcctagcctgggtaagaacagtgcatcagcttcagggcctttaattttctagttcctattactagtcttaattggccctttttttctccctaaaattatctattagacagcacccaaaagtaaaaaacaaatctagaaaattcaactcagttcccccccaaaaaaagagtcaggtgcacatttatttcccttatatctgctttattctacaaagaaatctacatatggtgatgagtaggcaatgtggcatagataatatgggaacagaaatgtgactcttgtgaatagatgcattaaaagatattttggactcacaagatagatttaacattttccaaaatgtacaaatttaagtgtgccgtcagttttcttaactttagaacagaagaagcaatcatttttataagttttgccatcagatccacaaattggatcatacatatgatgacaaaatctctgttgtcctggtggtaactttttataatgactgcagtcaaccatctgtttcgtctgtttggcacattctataccttgtaaatgttcaggttgcgttaagcccatgagtctcctgggttcattgtgttctcctgagctgcttggtggagttttataatgaaaacaatgatgagaaggattcataaagaccataaagatgcaaatgctgattgatcacacagagagacaaatctcaatgaaatcacttcttctccaatacctaaccttcaaaaggtaaaattttaaaaacaaatttacttcacattcatatgacggcaagttagcagcttcccatgtgggaatgatttactcttcctaagaataaagaaggaaagaaagttaataaagttaatatatatgtcattgtaagaaatacttataaattccattgacattaaacagtttataatgaaaaaccagtcttttatcatcagcatcacacttcagtgggaactcatttgaaccatttctgtttttagattattgccatcataattcttaataatatacatctattgccttacaagctaaaattatttgttgactcccacctatggaggaaaaaagtattaatttacatttccttttcattcatcccagtttttgataggcatatcatgactttttaaaattctgcttgttaactttgtaacctaaagtaatgtactttagtcactatttctat

SEQ ID NO: 15801 - RNA, 9702 nt, Homo sapiens
  source 1..9702: mol_type = other RNA
gctgggattacaggcatgagccactgtgcctggtcctaaactctaaacttcttttcttatgagctcttcttttcttttacaagtgctctttcttgaaaagaccattgtaaaggaggtcataacatgggatgtcaattcacatagatgcaccaatgactataagagaagcctccctagcttttgttttgagacggagtctcgctctgtcgctaggctggagtgcagtggcgcaatctcggctcactgcaacctccgtctcccgggttcaagcgattctcctgcctcagcctcccgagtagctgggactacctgcgcacaccaccacgcccagctaactgttgttgtatttttagtagagacggggtttcaccatgttggccaggatggtctcaatctcttgacctcgtgatctgcccgccttggcctcccaaagtgctgggattacaggcgtgagccactgtgcctggccaggcctccccagctttaagcaaagctgtgaagttaacagaatgattctaaatatctgcttgcttagaaaaagaaaaaaaaagtcatgtgaatccattggtcagaaaaaataaatatctacttgctacaggacaatagaatctaaaggcaatcatctaaatcactatcaatcaccctcccccagtctcctaaaatataagcaattagcaatgttcattatagtaggcatattatttttaagtcaaatttctaatggagttgtattcttctgtacttaagaagtaatcttgtagcacatatcgggctctttatatgtagagaagtatatgaccaatttactagctttagtgtaatttcacctcattacagaagttatagaggtgtgtataacatcacacctatgatttatttgatactaacttctggatatggaaaacaatatttaaaattttgaccactgcagagtgtaatataggacatcagttattttaggagttgctctttaaatgtggaaacatgatctcaatgtattgggccttcttttgggctgttttaagtaaaatttggctctgggaagaggcatcactgagttctttaattgtgagtttctgcagtttggcagttttatatcagaagttcctcattgtcataaaggcagatggtgaagctctgtcacataaacagcaatgctttcactgtgctgttcatcttgggaattttaaatctgtgaactaccatggaacaggtgaaaagtgggctttaatgaacccttaggttcattaggaaactaagcgaaaaggagagacttaccactggttccctcacatgcttttattcaggtctcatgtaaataatttgctttaagatagaatgaaatttgtgtgactatcaagcagtcagtttactgcatttccaagattgaggctgttatgttattttgctttctttttaaccacatcccggatgccagatttttatttttttaattgaggcagaaggagatgaggttgttgaagctacatcaaacctaaattagaacagtaataaaacgagaaatccaaaagaataaaagctgaatgatccatagagcccttgaagaatgtttctgtcagctattaatactgaagacagttgtctgatgaaataaggctatcagagtactttgggcaagttgattgacttcttgggagctttgcttatttatctacaaaataaataaggggtctaaaattacaaaagctcaagttacatatatatatttttttttttctttttttttttttgagacggagttttcactctcattgcccaggctggagtgcaatggtgtgatctcagctcactgcaacctctgccttccaagttcaagtgattctcctgcctcagcctccccagtagctgggattataggcatgcaccaccatgcccagctaattttgtatttttagtagagacggggtttctccatgttggtcaggctggtcttgaactgacctcaggtgatctgcctgccttggcctcccaaagtgctgggattacaggcatgcgccaccacgcccagcctctttccctttttctttataggcggtgttcaatagcatatcatgttacacatatcttcagagcccttttcctgttttaaggtcccattcctacctgccttcaagggacatcctcctgggttaaacatgctgcccttagtcactgtcggtaatccattgtgtcactggaggacaagccacccacaggtttctcctccttggtttggatactttctgaggtcaagagctgagaaggtgatgtaagtcctcggggctgtttagttgacttggtgagcttcttgagttcacttgcgaaagaaatgcctttctttttatcttctcgagatgcctgcacctgctcctttagcttaaggatgaattttcctgcacctttccacttgctttgggcttgaaacacacactcctgatccagaaggacccgctgagaggactttggtgtggtagtcttcttgttggtagtgtctttcaccacctcttccaaaagcacatagtcgcttggattggggttgctcaggatgctgtaggaatatttggctttgcataaggtctgctgaatgacatcctgtgcagtgctgacgcggggtgctttgatgactgttcgaggttgctctggagaaacatcatgcacttggacaaagaaactctcctcctctgagctcaagatcacctctttgtcatcttgaacaatgtttttctcttctaggttttcctgctgggtttttaagacaatcctgcccatgtatccctcttctggaaaccagctgcttaaaatttgcatgatctcctcttctggaccaatggctctctggaatggttgtttcctacattcattcttttctttagatataaaatatttttcttccatcaaaaaatagtctgtggtaacaggtttgatgtcttgttcatttgtcagaatttgctgcagaagctgctttgccttggtgcctccattaatagtgaaaacggtaaagggctctggccctgggaccccatgcaccgtgactctgtgagtctgcaaacattttctttcttctgtattaaacatcgaagaggctgacatggtattgccagaggaattttcttccatccttctgctgttaatgaataaactagaaatctccaagacttcattgtgaaggtttcgcagctgaagatgtcgatatcctcgttttaaagctttcagtggaatgattctctgagcagttaccgctgaactattgttttccacaactgcaaaacgaagaaatacaagatcttcgaagtgaacgtggaacagaaactgctcgttccacatggggttcagggtgtttcgatggatgggctttgtgcggaaatggcagctgtccagaggcatgcccaggacgtcgacttcaatgcacgggcttcccatgctattactggggcacacattctgaccagagacaatagttaaagaatagactgcaggatccatgctgtccagatctctttctagtggagaaaacttctgatacatggggcagttcttgtcccacagaactggaggtttcaatacataaccacaaccaccatttgcctcaaacattgcagcatttaaatgtaaagggagatcatcagtctggtagttgagtgccacaagctgtatcccatggagccagaacatgagggggttcgggttggaagagtcgatgcgggtggcagcagggtaagttctcagcagctgacaggcggtgtgctgggtcagtttctgagaatacctgcgacacagacgtttggcggcattttcattcagcgacgagatatgataacatttgggagttctaatgatagcactgagggacgtggttgggttgagaggggaagaagattcctcccaggtctgtcgaatgccttcacaggaactttttccagatgttttgttaaatgatgctgtctcccctgggctcattctgcccggattgttgccaaaaatggacttcctgcttttcctttcttttcctctgctagagccagatgcatttagagttgacagtcctggaaattttactgcttgacaatagattacaaggtcagaaagctctggtgcaatctgtctgctttcctttttattctgatcaagataaaattcttctcccagttccatatcataaacctttcctttgttgcaagcagagttatctgctttctttatcctctttgggatttcttcattatattcaaactgaagcttgtcattacatgatttattttcaggtctgtcttccagaatgttgtcttcctgaccgttaggagcaggggaggcagtaaggacatctgcatcagaaagggattcatagtcataatcatattcgtcctcctcatcttcctcttcctcattattggcaggtcgggggttggcattcccaccattataagcctgcacttgcatagatgctaactgatgagccttttgctttaagatatccactggcgtctgatgggcttttagcttcttgtttttaagaagaactttctttctgagttggtcaggtgaaggaagcattggatcatctgagaaatcagtctcaaataagaatttagtcaccagcttttctccaaacacagtcttgaaaatttctgccatttttcgttgctgaggcaatgaacagtggttctcaatcgatatgatgattggcaggtcagagttgatgaaggcactgcgatcaatggcttcaaccacttccttgaaggggatcttggttgtcagcgtatgtccatgataaatgatgggcatcccatcgtctccgtcccagcagtccaattctacacttcgacagccttgcaaaaggacctggctgtagagttctaccgaggattctcctttgagctgatggcccgtgaggtaggtattgtgcgaagattcgatgtaatagtatgagaggggtagctgcagttctttaatgttctcctgtgactcatcattttttgaggcaaaattttctttatccatcagaaacctggcaaacccttcaaatgacattagtccctgatgacacatactgatgctaggctcgaacttctggatgatgctgaggatttcatcataagtgcagtgttctccttggcaattcacgaggaaatcgttgagctgaagtatgcccaccccaaaaatgcccagagatgtgctctcaatcccagtgccatttgtcacaatgcttgcagcagcaatggcatcagatatctgcctctggttgtccgatagctgctgtttactcttaatgaacaaccccaaatccgagacatttctggtcaacagatctaggtcaggctgaagatcgctggtgttttcatcaattgtcaggttggtgtagagtggggctgactcggagccagatcggttgcagggcactgcatagacatcaaacagatccttcaggtccttgcggctcctgacactgaatgatttgaacagctcaacaaattcaacaaaactcatgttgctatctgaaaccatgaagctctgaaatcccttcatgccgcctttgatccgcccgtgccagctactactgctccaagcactggatgggctcttgtttgaagaagacagcacaggggaggacactggcctgatgggagatgacgtcccggcagccaagttgggggacccagctgtggtcaaagagtgggctcttctggaagggagggggtttggagggttagcgatggcattcacctctgattcttcttgttcattaatgtcttgaggatcagaaccactccggcttcgacactctttgtgcatcttggcctttcgggttgccatctcatcgtcagttacctctccactctcacccctcatgaggattttcttctttttcttggtagtgcttatgcccagggtattgtttctctgcatattgggcttctcagcattctttgctgatgttccggggctggggtttcgagcactccaccgtctgccaccaaacaactccacagcgtgagccaaagttgggccttcataccgtccatcctcctgataaaggctgacgtactgtttccgcagccactgctgtctttggtcagggaatttcctcatctttctcacagctctagtgagttccaataatccgctgaagagcattttagctgtgtgctttggtgccacgaagtgcaataatctgttgtctgtggtctgaagcccatagagcaatgtcacaccagtctctgacaggaacatgctacccagtttgttctgaacacacacagtgtgtatatcaatgccagggtggcccatgtatacagccttcactgcaaaaagatccaagaccccttccgtcaggctacttaatccagcattacccagtagtgggaattttccaggctcagctgtgttattaagtacaccaagttttgctttactgctggctggggaggcagttgtgggctttacccaggtcaaggtgctattgtcgggctgaagctggaggaagcagcgggcagagaggtgtgtgtcctggtcgtagtggatgaccgtggccccctgcagcaggaactggtgcacatcggcttggatggacagcacgtaccaagggatgagctccgtcccatggtcgaaggccttctgtgagtcctctgaaccatgagagtcgtattctttggattgctcaaagatgtcattgtctgaatccaacaaatctccaattataaactgccatcggcttttatccttcaaggagcttttcctggagctgtttccttcactggggctgtcctcctcgtctgtctccagacttcgattgcagctccggatgacctgaaagatgctgttgacagtggactccttctccgaattctttaagccattttgtcccactcgttgtaagaaattatcttgtccactgtaatctgctacaaactctaaagtttcttcttgggaattgtaccgcgggcaaagcttcatgagaccggaggcgccgtcaagcacttcacagagctccttcagaaacaccccacagaatggaaccaccttacagccagggatgtgcagggcacgtgtcaccacctttctgtactcacaagaggactcatgctgggccatagcatccttcaggctcctcatggtctcaatatcagactggtccatgaactgccacatttttaaaacttttcttgacctgaggccagccaagaactccatgacagcgttgtagttgcccatgttccagcagcatttggccacatgcaccaaatatgaaaagacttctcgcttctcctccatggagcctgccgtgaggatcagccatgtcacccaggagctcacctcattaaacctcatcaccagatcttcaagggcattgtgctctccattctgagtggtaagaatcgacgctgagatggatgctttgaggcagggcaaggagctctggcattcaggagtgcccaagtcccgtgttaagaagcaaaggtagtcgactggcaagaccctgcggtaaatagtctgctcttgctccatcaggatgctggcgacttcctctgggaactggatgagaggctgcagatcgatcagctccttgctgatcccagctgaacttgaagggagggcattggaattggccacagaggggcctggctggcgttctttcagcatcattcgtccagtggatcctccaaaagtactgagaaggccacttcttgctcccaaagacgtggttgcttctaggagagaaccggtgatgtactgcgatattgaagtcctttggagggtggcgcgatactcacatacagtgtctcggacacattgctttaagcatggaccaacgcttatccttccatgggctgtctcggaggctgggagcttggtgaggaaatggagtagagatccaactgtattttctgtttcttctcttctcactgcattgtagataggataccactgggcttctgacagacgttggctcccatcttgccttatctccactgttgacgggggttccattactctcccacaaggcagtaagggaccatttctcttctgatctatgtaactccatgcagtcagcccaatgtggccagaaggcagagttctcacaattgctcttgttccagtatacacagatttcttaacttctctgtcatttttacagaatctcctgactaacaaagtggatcgctcctttttgcttttaaaagcgtcttcttctacatcatcacaattatcagggaagtcctcaaaatggctcaaaaaggtcttggcagcttgactgtcagtaaagtctttcctacaaaagctatcacctgaatataccatgtcaaccttctcacaagagccttcaaagcaaaagtatttatcattcaaggtgtcacaatgatcacactgcagctgctcattcttattatcacaatttttggccaattccatcagtttacaggtatatgccacatagtttttcttttgcttctcctcacccccaggtagtggtacacaatttccacaatcgtctaaaattaagttttctgatagggtacagaaagtgtctgacattcttctgtcaacttcataatgaaaatgaaatactgcccttctgctgtcagggtgtgctctgcctgtctctatgatcactgactgatttcctaaaggactaatgcccatggaaggtctgtctagttccagttgaattccagggaacacctttctttccagtggagaaggaattccagtttctaaacacaagtcttcctcagcaacagagttgtacatttcataaaattgtctctgaggaaggccatgctgatggtttctcaatatgttgttgcagttaatgttaaggtttttcgcagaatctggcatgattttctcccaacatttttcattactgttctcatcactcactattttctccctcgctattgagagaatctttggcaagttgcttccagaaggttcttctttaagtttgttcagttgtgagatggtatgagaagtctccccacttcgtctgacagtatgtgcttttgaaatattgatgtctgagaccttttcactactttcatctgcagccgactgggcagaaaccacttttctctgagtcacaggtatgagaacagaagctgtcatttcttcagaagtcatcttggactaacacacaggttttgactattgctctatttttcctccctggtgatcatgtcaaggttttaataaaatgactgattattacaacaatctcagatacacaagtcctcccaaagaacaaagggataattcctttcattcaggagcattaagaggcaaataaattttcttagttataacttcctatcatgaatatatattttttctagatcagggttttaaggtggtagatcaattttccttcctctgttacctgaagcaaaattttttgaagacttttactcgggattgcactctgcaacttctgatccatcactgatttgcaatgattttaaaatccagtttgaatgattcctgtttcctcttggctcctggcgagtctcgccggcgtccccaagcgcagcgtccctctgggaccagccgtccgcgcgcctgtcgctagcggcgtcgggtgtccccgctactgtgtgtcagctgcagagccgatgcccaggaacgcgcaggagccaggcaagtgcccgagaggcagagcccgggaggcagagcccgggaggtagagcccgggcgcgccgccgctgc

SEQ ID NO: 15802 - RNA, 1296 nt, Homo sapiens
  source 1..1296: mol_type = other RNA
gctgggattacaggcatgagccactgtgcctggtctggattacatcttaacctacaatatttcatgaagttaatgattttaaataaaaggaaatcaagtaacatctgaatttctaagtctaaatacatttagatgatagtgactcctgcaactgtttcaaaattattggaaaatatgtcattttcttgaaatgaacttggtattaaaggcagcaaatatgtctttataaggagtttctgaatctgacttggtcgatggtattcggcaaagttggcgaaatccaggagaacgcagcagcaaattctgtgaaaggcccacgaagctggagcataaccagtagagaacaattgatcactgagggtaccgttgcagcaattggtatcatcaacaccgacattgcacggacaaagtacgtaatatacgtctgaaaacgagacattccaattttttgtagagcacaaatctccactattaacaaattgatgacgccaacagagataggcagaatccaagtggagtcgggtgcagtgaggtcaggaaaccacagaattccaccagtagctaactgttcctgaacagaaaaacctgcttctgaatgtgctgcccccgtgcttaaattccggagagcaaaagacatgaagatccacattggaagctgaatccaaaccaacacagtggctttgaaagggtggcagttatctcgcacatatagctctgaaattagcctcctcatattctttagataagtgagcctggcatctcttttggaccaccccaactgatttgcacgaactgcaacttcttggttaagatgcctggcaatagtttttatttctggctgcaaattttccaccttggccaggatgtagtgctggtaggctgccaaaggcagcgtgacagcaccccgtaaggccacggtggagagcagaatgctgccccaccagggcaggcccgtggcggcgtgcacgccgagcagtacttcctccgcaacccgcaccggcgaagacgcggccagggcctcgtaccagccgttcgcatgtactgcagagactggtgccactgcccacactgggagagtggggcgcttggcgccgctcgtaggaaccggcgcaagcggcaggtccctagcccaaagctgcagggcagggagcggccgcagccaccgaccgccgagccggcacagcatttctgcaccacggcggagcccagatcccgggcctcacaatccagcggacatacaccggccagccaaggctgatacgcgcacgcgccagcaacagcgggcataaagcgcat

SEQ ID NO: 15803 - RNA, 1293 nt, Homo sapiens
  source 1..1293: mol_type = other RNA
gctgggattacaggcatgagccactgtgcctggtctggattacatcttaacctacaatatttcatgaagttaatgattttaaataaaaggaaatcaagtaacatctgaatttctaagtctaaatacatttagatgatagtgactcctgcaactgtttcaaaattattggaaaatatgtcattttcttgaaatgaacttggtattaaaggcagcaaatatgtctttataaggagtttctgaatctgacttggtcgatggtattcggcaaagttggcgaaatccaggagaacgcagcagcaaattctgtgaaaggcccacgaagctggagcataaccagtagagaacaattgatcactgagggtaccgttgcagcaattggtatcatcaacaccgacattgcacggacaaagtacgtaatatacgtctgaaaacgagacattccaattttttgtagagcacaaatctccactattaacaaattgatgacgccaacagagataggcagaatccaagtggagtcgggtgcagtgaggtcaggaaaccacagaattccaccagtagctaactgttcctgaacagaaaaaccttctgaatgtgctgcccccgtgcttaaattccggagagcaaaagacatgaagatccacattggaagctgaatccaaaccaacacagtggctttgaaagggtggcagttatctcgcacatatagctctgaaattagcctcctcatattctttagataagtgagcctggcatctcttttggaccaccccaactgatttgcacgaactgcaacttcttggttaagatgcctggcaatagtttttatttctggctgcaaattttccaccttggccaggatgtagtgctggtaggctgccaaaggcagcgtgacagcaccccgtaaggccacggtggagagcagaatgctgccccaccagggcaggcccgtggcggcgtgcacgccgagcagtacttcctccgcaacccgcaccggcgaagacgcggccagggcctcgtaccagccgttcgcatgtactgcagagactggtgccactgcccacactgggagagtggggcgcttggcgccgctcgtaggaaccggcgcaagcggcaggtccctagcccaaagctgcagggcagggagcggccgcagccaccgaccgccgagccggcacagcatttctgcaccacggcggagcccagatcccgggcctcacaatccagcggacatacaccggccagccaaggctgatacgcgcacgcgccagcaacagcgggcataaagcgcat

SEQ ID NO: 15804 - RNA, 1263 nt, Homo sapiens
  source 1..1263: mol_type = other RNA
gctgggattacaggcatgagccactgtgcctggtctggattacatcttaacctacaatatttcatgaagttaatgattttaaataaaaggaaatcaagtaacatctgaatttctaagtctaaatacatttagatgatagtgactcctgcaactgtttcaaaattattggaaaatatgtcattttcttgaaatgaacttggtattaaaggcagcaaatatgtctttataaggagtttctgaatctgacttggtcgatggtattcggcaaagttggcgaaatccaggagaacgcagcagcaaattctgtgaaaggcccacgaagctggagcataaccagtagagaacaattgatgagggtaccgttgcagcaattggtatcatcaacaccgacattgcacggacaaagtacgtaatatacgtctgaaaacgagacattccaattttttgtagagcacaaatctccactattaacaaattgatgacgccaacagagataggcagaatccaagtggagtcgggtgcagtgaggtcaggaaaccacagaattccaccagtagctaactgttcctgaacagaaaaacctgcttctgaatgtgctgcccccgtgcttaaattccggagagcaaaagacatgaagatccacattggaagctgaatccaaaccaacacagtggctttgaaagggtggcagttatctcgcacatatagctctgaaattagcctcctcatattctttagataagtgagcctggcatctcttttggaccaccccaactgatttgcacgaactgcaacttcttggttaagatgcctggcaatagtttttatttctggctgcaaattttccacctagcttggccaggatgtagtgctggtaggctgccaaaggcagcgtgacagcaccccgtaaggccacggtggagagcagaatgctgccccaccagggcaggcccgtggcggcgtgcacgccgagcagtacttcctccgcaacccgcaccggcgaagacgcggccagggcctcgtaccagccgttcgcatgtactgcagagactggtgccactgcccacactgggagagtggggcgcttggcgccgctcgtaggaaccggcgcaagcggcaggtccctagcccaaagctgcagggcagggagcggccgcagccaccgaccgccgagccggcacagcatttctgcaccacggcggagcccagatcccgggcctcacaatccagcggacatacaccggccagccaaggctgatacgc

SEQ ID NO: 15805 - RNA, 1249 nt, Homo sapiens
  source 1..1249: mol_type = other RNA
gctgggattacaggcatgagccactgtgcctggtctggattacatcttaacctacaatatttcatgaagttaatgattttaaataaaaggaaatcaagtaacatctgaatttctaagtctaaatacatttagatgatagtgactcctgcaactgtttcaaaattattggaaaatatgtcattttcttgaaatgaacttggtattaaaggcagcaaatatgtctttataaggagtttctgaatctgacttggtcgatggtattcggcaaagttggcgaaatccaggagaacgcagcagcaaattctgtgaaaggcccacgaagctggagcataaccagtagagaacaattgatgagggtaccgttgcagcaattggtatcatcaacaccgacattgcacggacaaagtacgtaatatacgtctgaaaacgagacattccaattttttgtagagcacaaatctccactattaacaaattgatgacgccaacagagataggcagaatccaagtggagtcgggtgcagtgaggtcaggaaaccacagaattccaccagtagctaactgttcctgaacagaaaaacctgcttctgaatgtgctgcccccgtgcttaaattccggagagcaaaagacatgaagatccacattggaagctgaatccaaaccaacacagtggctttgaaagggtggcagttatctcgcacatatagctctgaaattagcctcctcatattctttagataagtgagcctggcatctcttttggaccaccccaactgatttgcacgaactgcaacttcttggttaagatgcctggcaatagtttttatttctggctgcaaattttccaccttggccaggatgtagtgctggtaggctgccaaaggcagcgtgacagcaccccgtaaggccacggtggagagcagaatgctgccccaccagggcaggcccgtggcggcgtgcacgccgagcagtacttcctccgcaacccgcaccggcgaagacgcggccagggcctcgtaccagccgttcgcatgtactgcagagactggtgccactgcccacactgggagagtggggcgcttggcgccgctcgtaggaaccggcgcaagcggcaggtccctagcccaaagctgcagggcagggagcggccgcagccaccgaccgccgagccggcacagcatttctgcaccacggcggagcccagatcccgggcctcacaatccagcggacatacaccggccagccaag

SEQ ID NO: 15806 - RNA, 1250 nt, Homo sapiens
  source 1..1250: mol_type = other RNA
gctgggattacaggcatgagccactgtgcctggtctggattacatcttaacctacaatatttcatgaagttaatgattttaaataaaaggaaatcaagtaacatctgaatttctaagtctaaatacatttagatgatagtgactcctgcaactgtttcaaaattattggaaaatatgtcattttcttgaaatgaacttggtattaaaggcagcaaatatgtctttataaggagtttctgaatctgacttggtcgatggtattcggcaaagttggcgaaatccaggagaacgcagcagcaaattctgtgaaaggcccacgaagctggagcataaccagtagagaacaattgatgagggtaccgttgcagcaattggtatcatcaacaccgacattgcacggacaaagtacgtaatatacgtctgaaaacgagacattccaattttttgtagagcacaaatctccactattaacaaattgatgacgccaacagagataggcagaatccaagtggagtcgggtgcagtgaggtcaggaaaccacagaattccaccagtagctaactgttcctgaacagaaaaaccttctgaatgtgctgcccccgtgcttaaattccggagagcaaaagacatgaagatccacattggaagctgaatccaaaccaacacagtggctttgaaagggtggcagttatctcgcacatatagctctgaaattagcctcctcatattctttagataagtgagcctggcatctcttttggaccaccccaactgatttgcacgaactgcaacttcttggttaagatgcctggcaatagtttttatttctggctgcaaattttccacctagcttggccaggatgtagtgctggtaggctgccaaaggcagcgtgacagcaccccgtaaggccacggtggagagcagaatgctgccccaccagggcaggcccgtggcggcgtgcacgccgagcagtacttcctccgcaacccgcaccggcgaagacgcggccagggcctcgtaccagccgttcgcatgtactgcagagactggtgccactgcccacactgggagagtggggcgcttggcgccgctcgtaggaaccggcgcaagcggcaggtccctagcccaaagctgcagggcagggagcggccgcagccaccgaccgccgagccggcacagcatttctgcaccacggcggagcccagatcccgggcctcacaatccagcggacatacaccggccagccaag

SEQ ID NO: 15807 - RNA, 1246 nt, Homo sapiens
  source 1..1246: mol_type = other RNA
gctgggattacaggcatgagccactgtgcctggtctggattacatcttaacctacaatatttcatgaagttaatgattttaaataaaaggaaatcaagtaacatctgaatttctaagtctaaatacatttagatgatagtgactcctgcaactgtttcaaaattattggaaaatatgtcattttcttgaaatgaacttggtattaaaggcagcaaatatgtctttataaggagtttctgaatctgacttggtcgatggtattcggcaaagttggcgaaatccaggagaacgcagcagcaaattctgtgaaaggcccacgaagctggagcataaccagtagagaacaattgatgagggtaccgttgcagcaattggtatcatcaacaccgacattgcacggacaaagtacgtaatatacgtctgaaaacgagacattccaattttttgtagagcacaaatctccactattaacaaattgatgacgccaacagagataggcagaatccaagtggagtcgggtgcagtgaggtcaggaaaccacagaattccaccagtagctaactgttcctgaacagaaaaaccttctgaatgtgctgcccccgtgcttaaattccggagagcaaaagacatgaagatccacattggaagctgaatccaaaccaacacagtggctttgaaagggtggcagttatctcgcacatatagctctgaaattagcctcctcatattctttagataagtgagcctggcatctcttttggaccaccccaactgatttgcacgaactgcaacttcttggttaagatgcctggcaatagtttttatttctggctgcaaattttccaccttggccaggatgtagtgctggtaggctgccaaaggcagcgtgacagcaccccgtaaggccacggtggagagcagaatgctgccccaccagggcaggcccgtggcggcgtgcacgccgagcagtacttcctccgcaacccgcaccggcgaagacgcggccagggcctcgtaccagccgttcgcatgtactgcagagactggtgccactgcccacactgggagagtggggcgcttggcgccgctcgtaggaaccggcgcaagcggcaggtccctagcccaaagctgcagggcagggagcggccgcagccaccgaccgccgagccggcacagcatttctgcaccacggcggagcccagatcccgggcctcacaatccagcggacatacaccggccagccaag

SEQ ID NO: 15808 - RNA, 1188 nt, Homo sapiens
  source 1..1188: mol_type = other RNA
gctgggattacaggcatgagccactgtgcctggtctggattacatcttaacctacaatatttcatgaagttaatgattttaaataaaaggaaatcaagtaacatctgaatttctaagtctaaatacatttagatgatagtgactcctgcaactgtttcaaaattattggaaaatatgtcattttcttgaaatgaacttggtattaaaggcagcaaatatgtctttataaggagtttctgaatctgacttggtcgatggtattcggcaaagttggcgaaatccaggagaacgcagcagcaaattctgtgaaaggcccacgaagctggagcataaccagtagagaacaattgatgagggtaccgttgcagcaattggtatcatcaacaccgacattgcacggacaaagtacgtaatatacgtctgaaaacgagacattccaattttttgtagagcacaaatctccactattaacaaattgatgacgccaacagagataggcagaatccaagtggagtcgggtgcagtgaggtcaggaaaccacagaattccaccagtagctaactgttcctgaacagaaaaaccttctgaatgtgctgcccccgtgcttaaattccggagagcaaaagacatgaagatccacattggaagctgaatccaaaccaacacagtggctttgaaagggtggcagttatctcgcacatatagctctgaaattagcctcctcatattctttagataagtgagccttggccaggatgtagtgctggtaggctgccaaaggcagcgtgacagcaccccgtaaggccacggtggagagcagaatgctgccccaccagggcaggcccgtggcggcgtgcacgccgagcagtacttcctccgcaacccgcaccggcgaagacgcggccagggcctcgtaccagccgttcgcatgtactgcagagactggtgccactgcccacactgggagagtggggcgcttggcgccgctcgtaggaaccggcgcaagcggcaggtccctagcccaaagctgcagggcagggagcggccgcagccaccgaccgccgagccggcacagcatttctgcaccacggcggagcccagatcccgggcctcacaatccagcggacatacaccggccagccaaggctgatacgcgcacgcgccagcaacagcgggcataaagcgcat

SEQ ID NO: 15809 - RNA, 1275 nt, Homo sapiens
  source 1..1275: mol_type = other RNA
gctgggattacaggcatgagccactgtgcctggtctggattacatcttaacctacaatatttcatgaagttaatgattttaaataaaaggaaatcaagtaacatctgaatttctaagtctaaatacatttagatgatagtgactcctgcaactgtttcaaaattattggaaaatatgtcattttcttgaaatgaacttggtattaaaggcagcaaatatgtctttataaggagtttctgaatctgacttggtcgatggtattcggcaaagttggcgaaatccaggagaacgcagcagcaaattctgtgaaaggcccacgaagctggagcataaccagtagagaacaattgatgagggtaccgttgcagcaattggtatcatcaacaccgacattgcacggacaaagtacgtaatatacgtctgaaaacgagacattccaattttttgtagagcacaaatctccactattaacaaattgatgacgccaacagagataggcagaatccaagtggagtcgggtgcagtgaggtcaggaaaccacagaattccaccagtagctaactgttccttctgaatgtgctgcccccgtgcttaaattccggagagcaaaagacatgaagatccacattggaagctgaatccaaaccaacacagtggctttgaaagggtggcagttatctcgcacatatagctctgaaattagcctcctcatattctttagataagtgagcctggcatctcttttggaccaccccaactgatttgcacgaactgcaacttcttggttaagatgcctggcaatagtttttatttctggctgcaaattttccaccttggccaggatgtagtgctggtaggctgccaaaggcagcgtgacagcaccccgtaaggccacggtggagagcagaatgctgccccaccagggcaggcccgtggcggcgtgcacgccgagcagtacttcctccgcaacccgcaccggcgaagacgcggccagggcctcgtaccagccgttcgcatgtactgcagagactggtgccactgcccacactgggagagtggggcgcttggcgccgctcgtaggaaccggcgcaagcggcaggtccctagcccaaagctgcagggcagggagcggccgcagccaccgaccgccgagccggcacagcatttctgcaccacggcggagcccagatcccgggcctcacaatccagcggacatacaccggccagccaaggctgatacgcgcacgcgccagcaacagcgggcataaagcgcat

SEQ ID NO: 15810 - RNA, 840 nt, Homo sapiens
  source 1..840: mol_type = other RNA
gctgggattacaggcatgagccactgtgcctggtctgtgatctctagcatttcttaaaactgcatgtgaatcaacaattgtcttaaaataaaaatgtgtgtgtgtgtgtgtgtgtgtgtatgtgtgtgtgtgtgttttggaatgtcagtgagggaagtggatggagaggatgcagaggggaaaaggtaaggacttgcccaagttcacactgggtgatggagctacatactcaggctcataacctctgctttgagccaccaccccatctgacagaaaactgttatgaccttcacttctggaatttccccttcctctttccaaacaagccaagattacaaggcccatgctcttactcacacccagggtagggtgtgtgagttctgtacccatcagtaccacagataggaggggtccaagaaggctgggagccacatcaggtctgagtccttttagaggaattaacatagacattgagagacagatgctgtagctctgaaaggaccattgaaactgaattttccaagtgccattttccccaccacgtagaagtagtgtgccttaaccaagtatgtgtgatgtttaaacgtttgcgggacaaatggaacaggaacgtctatgtcaggaaactttgcctttgccactctctgtgttcaggtggagctgccctcaccccgggcaccatgggcggccacagaccagttctgtctagtgagggcccatctgctcctggccatagtgactaattcagtgatgggcacttgacacaagccaggtcaacaatatttgatttgggagttttgatggcccaaggcagttagagagctagatactagttggcct

SEQ ID NO: 15811 - RNA, 3724 nt, Homo sapiens
  source 1..3724: mol_type = other RNA
gctgggattacaggcatgagccactgtgctcagccaatctttacatggtatatctttctccatccttttactttttacatacttacgtcatttaaagtggacttctaatatatagcatatagttgggtcttgtattcttaaccaaaatgacaaactggcttttaaatggtgtttctagaacatttacctttaatgtaactgttaatatagttggatctatcattctattatttgttttctgtttttctcctttttttcttcattcctttttctccttttctgaattttttttttttttttgagagagggaattgctctgttgctcatgctggagtgcagtggtatgatctctgttcactgcaacctctgattcccaggctcaagcaatcctcctgcctcagcctcctgggtggctgggactacatgcacacatcaccatgtctggctaattttttaatattttgttttggagagatggggtctttccatgttgcccaggctgctaagtcctgggctcaaagaatctgcctgccttggcctctcaaactgttgggattacagacatgaacaaccgtgcctggctctttcctggattcttttgaattatttgaatatcttttggttttctatctcttggctttaaaaataactgtatatattttttgttttgtttttgtatttgagacagtctcgctccgtcaccaggctggagtgcaaaggcatgatcttggctcattgcaacctctgcctcctgggttcaagcagttttcttgcctcagcctcctgagtagctgggactacaggcacgcaccaccacctccagctaatttttgtatttttagtagagatggggtttcaccatgttggccaggatggtctcgatctcttgactcatgatccacctgccttggcctcccaaagtgctaggattacaggtgtgagccactgcgcctggccaaaaataactatatacttttaataatattcttaatgattaaggattccaatatatgtatttaacttttaaaaccagctaagaatattttatcatttcaaataaaatgtggggaactttcaacaatacaggtccttttacattccaccctttatgttgcagttgtcatgtgtattattatctacatacaccaaaaatcccaccatcaatgttacagtgtttgcttgcacccattatacatattttaaagaaattatgaagagtaaaaagtatatttatccatatatttactgtttctgttgctcttctttcattcctgaagttttgagtttccttctggtattacttcctttccacctgaagaattccctttagcatttcttttagtgcagctgcattattttcccttcttctgggaaggaattattttgcctgcattcctgaggaaaattttacagaatatagaattttgggttgacacttctttactttcagcatcaaaaaaatgttctactgctttctgaccgccatgatttctgatgagaaatccagtcattttagtcatttcgcctttatatatgtaatgtgtcatttttctttttcaatttttttttttaaggcagtgtctcactctgtcgcccaggctgtagtgcagtggcacaatctcggctcactgcaacctccacctcccaggctcaagcaattctcccacctcagcctcctaggtagctaggactacaggtgtgcaccaccatgcctggctaatttttgtatttttttttttttttagagatgggggctttgccataggctggtcttgaactcctgggctcaagcaatttgcccgccttggcctcccaaagtactggaattacaggcatgagtcatcacacctgcccacattttaaaatttttcagcaattaaaaatctttaattttcagcaagtaaatttggatgcatctcaatgtagtttttttgttgttgttgttgattttagtgtatcttgtttggggggtttcctgaacttcctgaatctttacattcatgtcttttgccaaattttaaagtttctatcctttatttttttcaatattcatctgcagcagtatcttcctcctgatctgggacaccaaagacataaatgttaatctttctgatattgtcccacaggtatgcaagtctgttatttttttcaatcttttttcctctctgtttcaaatgggataatatatcttgatcttgaccttttaagatcactattttatcatttccattcggcaaatgagtccatccagcaaaggttttaatttcaattatgtagttttcagtttgtacataaccgctttgtccttccttcctgccttctttcccttccttcactgtgaaacataatttagttttacttagaactatattatgaacatctttctaggtaagtacataccaatttagttttattctggtaaaatacatgtaacataaaatttaccatcttaaccatttttggtatacagttcagtagtgttaagtacattcacattgttgcgcaagcagtctctagagctcttcttgccttgcaaaactgatactccatatccattcaacaactctccattccccactccccatggcactttcttgtagcttctatttttctgcagataatttttctttcatttcaagagtgttctctcttcttactgctctcttattgctattatgtacttttcagactcctagttgtgttttctttcaagggtttttggttgtaatctttgggaaagataaagtgatatgtgctgcttactccatctgaactggaaattaaagtctgaactccttttttaattaatcaatcaattaattaatttttttgagacagggtctcactgtgttgcccaggctggagtgcagtagcatgatcaaggatcactgcagccttgacaccctgggctcaagtgatccttccacctcagacctgtgagtagctatacctggaacttggctgtaatagctgctttgaagtcactgtctgataggtttaacatctgaatcattttgggactggcttgtttcttgcaagttggtgagattttcctggttccttatatgttgagcaattttagattattcctgaatgttacatatattttacaagtctctgagtcttgttaaagtcctttggtgaatgtttactttgttgttttagctgccaattaacctggttggttcagatcataagtttggacatacctttagtaagctgtggctttagtgtcacttcagtttccaaaggttttgcagtgctacttggatctgcctcacatgtgcatcacccaggtggtcattctggtggtagtctacaccacagccagttctcagagcctttggtatattgctttgggtcagctccatgcatgagcagctgggggtggagccaaggactttatacacagctttttaggaacttttccttgagcttcctcttttctgtgatttcccccatactctcctgctgccaagagcctctttttctgcttgtgtggttttactacactgggcaaatatcagtctatgcagaactgtccccactcaaagataaggaaaatgatggtatgcaacctatgcaaaaataatttttataattaagggctataacatgaaaaagataaatgcagaatatacacttgaagctcggtgtgatggcacacacctataatccccgcatttcgggaggctgaggcaggagggctgtttgagcccaggag

SEQ ID NO: 15812 - RNA, 3618 nt, Homo sapiens
  source 1..3618: mol_type = other RNA
gctgggattacaggcatgagccactgtgctcagccaatctttacatggtatatctttctccatccttttactttttacatacttacgtcatttaaagtggacttctaatatatagcatatagttgggtcttgtattcttaaccaaaatgacaaactggcttttaaatggtgtttctagaacatttacctttaatgtaactgttaatatagttggatctatcattctattatttgttttctgtttttctcctttttttcttcattcctttttctccttttctgaattttttttttttttttgagagagggaattgctctgttgctcatgctggagtgcagtggtatgatctctgttcactgcaacctctgattcccaggctcaagcaatcctcctgcctcagcctcctgggtggctgggactacatgcacacatcaccatgtctggctaattttttaatattttgttttggagagatggggtctttccatgttgcccaggctgctaagtcctgggctcaaagaatctgcctgccttggcctctcaaactgttgggattacagacatgaacaaccgtgcctggctctttcctggattcttttgaattatttgaatatcttttggttttctatctcttggctttaaaaataactgtatatattttttgttttgtttttgtatttgagacagtctcgctccgtcaccaggctggagtgcaaaggcatgatcttggctcattgcaacctctgcctcctgggttcaagcagttttcttgcctcagcctcctgagtagctgggactacaggcacgcaccaccacctccagctaatttttgtatttttagtagagatggggtttcaccatgttggccaggatggtctcgatctcttgactcatgatccacctgccttggcctcccaaagtgctaggattacaggtgtgagccactgcgcctggccaaaaataactatatacttttaataatattcttaatgattaaggattccaatatatgtatttaacttttaaaaccagctaagaatattttatcatttcaaataaaatgtggggaactttcaacaatacaggtccttttacattccaccctttatgttgcagttgtcatgtgtattattatctacatacaccaaaaatcccaccatcaatgttacagtgtttgcttgcacccattatacatattttaaagaaattatgaagagtaaaaagtatatttatccatatatttactgtttctgttgctcttctttcattcctgaagttttgagtttccttctggtattacttcctttccacctgaagaattccctttagcatttcttttagtgcagctgcattattttcccttcttctgggaaggaattattttgcctgcattcctgaggaaaattttacagaatatagaattttgggttgacacttctttactttcagcatcaaaaaaatgttctactgctttctgaccgccatgatttctgatgagaaatccagtcattttagtcatttcgcctttatatatgtaatgtgtcatttttctttttcaatttttttttttaaggcagtgtctcactctgtcgcccaggctgtagtgcagtggcacaatctcggctcactgcaacctccacctcccaggctcaagcaattctcccacctcagcctcctaggtagctaggactacaggtgtgcaccaccatgcctggctaatttttgtatttttttttttttttagagatgggggctttgccataggctggtcttgaactcctgggctcaagcaatttgcccgccttggcctcccaaagtactggaattacaggcatgagtcatcacacctgcccacattttaaaatttttcagcaattaaaaatctttaattttcagcaagtaaatttggatgcatctcaatgtagtttttttgttgttgttgttgattttagtgtatcttgtttggggggtttcctgaacttcctgaatctttacattcatgtcttttgccaaattttaaagtttctatcctttatttttttcaatattcatctgcagcagtatcttcctcctgatctgggacaccaaagacataaatgttaatctttctgatattgtcccacaggtatgcaagtctgttatttttttcaatcttttttcctctctgtttcaaatgggataatatatcttgatcttgaccttttaagatcactattttatcatttccattcggcaaatgagtccatccagcaaaggttttaatttcaattatgtagttttcagtttgtacataaccgctttgtccttccttcctgccttctttcccttccttcactgtgaaacataatttagttttacttagaactatattatgaacatctttctaggtaagtacataccaatttagttttattctggtaaaatacatgtaacataaaatttaccatcttaaccatttttggtatacagttcagtagtgttaagtacattcacattgttgcgcaagcagtctctagagctcttcttgccttgcaaaactgatactccatatccattcaacaactctccattccccactccccatggcactttcttgtagcttctatttttctgcagataatttttctttcatttcaagagtgttctctcttcttactgctctcttattgctattatgtacttttcagactcctagttgtgttttctttcaagggtttttggttgtaatctttgggaaagataaagtgatatgtgctgcttactccatctgaactggaaattaaagtctgaactccttttttaattaatcaatcaattaattaatttttttgagacagggtctcactgtgttgcccaggctggagtgcagtagcatgatcaaggatcactgcagccttgacaccctgggctcaagtgatccttccacctcagacctgtgagtagctatacctggaacttggctgtaatagctgctttgaagtcactgtctgataggtttaacatctgaatcattttgggactggcttgtttcttgcaagttggtgagattttcctggttccttatatgttgagcaattttagattattcctgaatgttacatatattttacaagtctctgagtcttgttaaagtcctttggtgaatgtttactttgttgttttagctgccaattaacctggttggttcagatcataagtttggacatacctttagtaagctgtggctttagtgtcacttcagtttccaaaggttttgcagtgctacttggatctgcctcacatgtgcatcacccaggtggtcattctggtggtagtctacaccacagccagttctcagagcctttggtatattgctttgggtcagctccatgcatgagcagctgggggtggagccaaggactttatacacagctttttaggaacttttccttgagcttcctcttttctgtgatttcccccatactctcctgctgccaagagcctctttttctgcttgtgtggttttactacactgggcaaatatcagtctatgcagaactgtccccactcaaagataaggaaaatgatggtatgcaacctgtagtctcagcttcttgggaaactgaggtgggaggact

SEQ ID NO: 15813 - RNA, 2121 nt, Homo sapiens
  source 1..2121: mol_type = other RNA
gctgggattacaggcatgagccactgtgctcagccctaaaatattgttagagaacatttacagacataaagatgagctcagtctcatccttatcaatctcctaaaaggaaaatttaagatctagtacttataatcctgtcctcaaagcaaacctaaaaataactgtctctctgatttgttttacagaatcatttatagttgtgtctgtcaaatagcaagaatcattcctagccagtgatgtggttatcacttatcttatgtgagggtaaacctgcaatatcttagagtcctttctaaaattatacagaagtcaaaataacctttccaaaaaggagtactaaaaaactgtcactgatagaaaacatcaactgtatgccaaagtactaaaaaacaggcaatcattccatttcagttgtattcacctattttcatcagtaggcagggcagtgctatcagaagagtaggctgcccttctatgacgacagaagctgttcctgatacttagttctgccttgcacatagtagactcaggtatcagtaaaatgaatgaatgaattatgaaatacactgactggtgagtcagacgttttttaacattccaggaaaaaaaagaaggctgaaattcctaatgaaaaaaggatgtctcattgagagatttttgcattactctttctgtatacgaaagcttgttgtttagataaattaccacaacacaggactttcacatacctgtctttattttgcttttatttgtgatttgatttaaataaataagaaggttcacacaggttaataaaaagacaagcaagtttgttgtatggctgagaaataatatgctctcttggtgtatactgatggcattatcggataacaccatgaggaccctcctcttcctcatttcctgggtcagtcctggtcagtgcttcttccgcctagtgctccttttgtatcacttatgtacactggatggagagaaaagaactcttctatgccttagtcaacatagatagcagcaggtgagaaaaagagctgatttctgatgtaacagaagcagactgactcctgctagctccagatacaaaatgctctacaggatgacttactgtaagtcactactgataagttgtttgcgtgactgctgggagacagatttacagagttctgtgacagtctattctggtcttgctcagtttggtcaggagcaggagcccatgtgtcaggagcaggagcccatgtgtttttgctgatcgagtcgaactcggagcccccagggtcttttaagttgttttcatctgattgtcggttcttttggggagaggcaaaagggttgaagtttccttctaccttacgatgcggctgtgtgttgaactccgtttcaaaagatgacagctgctgcgttactcctaaaagtccacccacctccacactgagaatcacccagatgacatctccatagtagagtcctgtagcagtgcacatccgccactgtccctgatacattcctgctctgctggggctgcacatctggacgctgacatctgcaatctcttggggctctagcgatctcaccatcaccatgttcacatgtccaaattggtctcccccgacatatttaagacaaacccctggaggccaggcctctgccccagaattctggatccgccatgtttttacaaactgagtatccggaggtattgactccccttctcctatggtgacatcttcaacaaaggacatagagggcacactgatgtttgggctctcaaagtcataataggcgccaattgctgcttgtaggttccagttggtcatgtccaggaagaaggcgcaaccggcaggattgagctggaagccgagcagcctctggaactcggagatgagcacgtccttgtcggtggtgcccaggcagctgaacttctgcatcagctccgggtccaggtctacgtccatgccctccatggcggggaccggacacccgcttccccgcctcttcacaaccaagccgccgccgcgccgccgggcccggggacctggaggggggccgctgctagctagcttcgcgaccccgctcctttgaggtaggccccgggcctctcacagtctcataggggtaaactcact

SEQ ID NO: 15814 - RNA, 6619 nt, Homo sapiens
  source 1..6619: mol_type = other RNA
gctgggattacaggcatgagccactgtgctcagctggcatttgttatataacagaccattccttgaaaatgccaacaaaacaaaacttttcaccaccctaaccagaaaaatgaacttttttttctaaattgccctatttctgtcagtgattccaatctcctaccaaagaaacatttactctgaaataattaagtccttaaaactctgtgttgaattgattactcttccccgctttcagtcttctaaggcctgtctgttcctatcacatgtttctccaatccacccttactactctactgtgatgtcaacacaaatttctgaattattaaagaaacttccaaggaagtctcttttactccaatctctttaccctccccagtcaaagctgcagtaaaacctgtactttaagaagaaggctttcaggtcatttctcccttgtgagattatacaaagtttggatgcaaaataaaaatctaaaccaagaaggttgtgataagttcctcctttatgcagcctcatcacatctcctccttgacagtattaatatgctgtgcttatcttctcctccaacaccaggcccatccctacatttttccctcatggaatttattctcctcacctgctctattcttctttctcttctctgtgtccaattaagccaatgttcaagggtcatttcagagtgtacttcaagaccaagtgccctggtagttctagtcctttctctgcactccgtatcggtaagaatcacagaatgaactatggtcttctaattgtttttatacacacttccctgtactccaactagatacaaacaccgtgccttacactaccagccacgtggctggaccaggcaaggtaaagttggtggccaagggagaaggtctacaaacgcaccccaaacaaggatcccacccatggctttgctgcatcagcaaaaactctgatgaactaaagtcctcctccaaaaagacctagaggaaatatccaaatgaacagatcacttaacaatatgtagattatttaacagtaaaacaggcgattgccagagtaaatattttccatacgctacacaagccttaaaacattgaagttaaagctgaaaacattgacattaaagttggtttctatggatgtcaactacaactctgacagcaccattaataattcacatttcttagtttcttttggaatccagtcaactcctttctctagtttcaagaacccctaactccaagcacaactgtctgtgcttcaggtttcaactgcaaatagctagtttgtcagtacatgtcacattcattttttaattttctgtttagttacttaccaggctacacacaatatctgtctcaacattaacattattcataaccattttacctccccctcctcttgtgaacatgagaattattttaacacaccaaagagttaaaacagagacccagtcaattttaggtgtttggtaacaccctgccattttgtacaagaagtggctgtgaaccagagtctatttcagtggccaaattccatagtagaagtgagcttaaaaatactcaaggtcctaatgtgcttccagtctagaaggaccacatttgtaaggcattcctttggatcttgagtgatcataagcccctggaaagcaggtactactctctctctgcttcttgtttgttcaaaacaaactttttgggcacctaccatggtctatgtgctgtgctggacactgggaatgtaaagaggaacaaactacagttccttccctccaagaacttggtctacaagaacctagcaatgttgggtgcacagtagatatttaatacgtattaaatgggtatttccataaagagtccccataggttctctgggcccacgatgagaactcaaccattcatttcacaaatgataagtttgcagttgggccaaaaacctttaatttcaatgaaaccataacctgcaatggcttatgtcagagaacaacataaatatttgctttaagagctggtgccaagaatctcatgcaaactttaggcaaaatgttttagctgaggggtacttggctaaaaccagagggcttggaaggaggaaaatgtaatgcagagtctgctgaactttgacccatggcatcagtgaagtccaacaacttttcaagtcttggtcttctcatttgtaaaatggggacaatgcaaggctatgatttattcctcacaggaaaaaaagtcctctggaaatgtaaaagccgcattagagtaatgtttaataattcaagatgaggtctggaagaacatcaacagtctctcaccctctgtgcccaggcattttgaaagggcactgtgccaaagtccattagtgctgggaatacacatcagcaggaagccttttgcatcttgactccctttccattgagcccctgaaatcagatgcctaacaggaagataggaagctgaagtgttatgggaccccagctatcagtcaaacggttttcctaatgtctcctttttagttgttttgttttaaagaaagaattagctttcacaatcaaggttgctgtgattctaaaaatcccacaaaaatgcccgcttggaatgcctagcttttcaaggcttcaggtaacctgaaagtcctctgattcagatactggcagaacctgaacatgctgacagcttggattaatttgggggaaaggatgcaaggggcaataaaatattctaacttcagattcaaagaggcagcaatatggtgaagaaaagcacaaagttccaaaaccagactgacgttctctcccccaactgacttgtacattcagtgaattaactcagctgtgtatttccccaatatatcagcctggtgagagatgccataaacagacctgcaggcaaccctacagacatcccttatccctcccctcctccaggggtataaaggaaagctaacattaagtgaaagacataagtctagagctgcaatgtccatagtggtagtcaccaggaatgtgtgaatagccagcatccaatagatagctagtccaaattgagacgtgctatgtggataaaatatccaccagatcaaaaagactagtatggaggaatgtaaaatatttcaatattttatactgaatacatgctgaaataatattttgggtatattaggcttaaaatatataattaaaaataatttcatctgtttttttatttcttcatgtagctactagaaaattttacagtataggcaaggctctcaattgtagcccaaactgtatttttcttggacagtgctggctcagagcatcccagtttcacctggatcctttgaaaggacaaattgaacatatggaaatgcagtcaggctcacaaaacaaataacctcattttccatgaggtgaccttgacaccattgaaagaatgaagccgattacatggctgtcctctcacagttgatctccaagtacaagactgtttcttgtcaggctaaatgctctcttgcaatgatctgttttagataataccaagaaaagctctacagggtatgggtcaaagcacaggtactggagtcaggccgacctgggtttgaatcccatctctgccactttctagctgggtaatctcaggaatattatttaatatattaaggtgcctattctctgtaacaggacaatcagatttcttcacagagaaggggagggaagggttaacacagcaagggagatgaagaatcttgggcaccatgcctaacagacagcacttgagaatggtagccatctagtaaaattctagcaatcttatctgagcaccttccagaataatgatgaggtaggggagacggggatggggtgcaaaggagatgggaccacttgtccacagaccttggagtcagtgaattaaagccgaatcctcaggaacggtatttattccacacagtgcaacactgccctctagtgacaaagaggtggaaaagctttcagagcatgaggcaagcaaggaagaaaaatacatttttccaggctctaagacagtaagttctccaaatcagagagatcatatcaaagaataattttttctcatgagtcacctttaaagcagtgacatggagtatgaagagcaatattatcaagatttactaccaacccagaggttgtcactttgttaattatataatatctcaaataggaaaaacagtaattctctctagacatattaaatgtgacacctaaaaagaagaaagtctgagtgttccaggttactcgacattattctggtaggacagcacggaggtttaagattcatgtataacagtttgtaaaccagatttgatcacagatttggttaatgcaactaacaaggtcaaaacttaaggctgaactggtatacaaacttggaaggaatacttaccatttttaacctcttttctccttgcagagcacctaagtgaggctaacagtaccctgggttgttgtggggagtaaataagaaagaacaccgaaatgcccagcagagtgtctaacacacaagcagtaagtgttagctgctgctatttttgttgtttctgttgttccaactgccacaggcccaaatggaggaaaagccataagataaaataactccttttacttttttgggttaaaaccaaggcttacctagtttcatttcctgatgcatctaccaatcaaatgtatcattttataacaagaacatcttagcacaactttgatgtccctgagattataatgctaactgaagtttggtaatagtttagaattcagatactgatctttaataaggcagaaagatgatgctgtaatcaaaaccgtctgcagagacaagacgtgtcaccatttctatcgtaaacctactatggtcgttttaggcagtctctgcccatcttcattcttctcaattaacttggatgaaaaacataatactttaaattggaaattttttataataattttcctcacttaattttcatttttaatatagtgatctcacgtccaaacatttcccatttgatgatcaccgggtaaccatgtgaccccttaagccagtcccagacaactataatacatgctttctagtattgtacagttcttgtttcaatatcctgtagtcacttctatatccttgtcatggtatggtcctaagacaatccagccacagaatgtgtaacccagataaatcataccagcacaagcacaaaaccgaagaacttttggcagtgaggcctgcattgttaaaatcagcacattatatgcctggaaataacccaggtatctgatgactccaacccaaaccaagagcgtagaggttccaagaaaaatgctgcagagatcatagtttgtgagattcagccgttgatgaactcccactggtcggtgtcacacacaggccgcttgtacttctccaggaagaaatttagaaatctcttccgtaaccttagagcaagaacaatggatcttgtacacagaataagagatgccaagcaaatcacaatgacaaatgcatcaaacaccaggacatactgagcatttttctgagtagatccaaatatgttcaagtctttacattcttcaattttggcatcactgtcaaaatagattttgattttgccactgtgagctttattgtcaaagataatcgtattctgaaagacataacagtctggtaactcacgggaatgaattgtctgtaggtcaatgcctttaagatgaaaggagatttcaacctgtaagagccgataaaattccagtctgaagaatgatgagttcttccagtccggaggcttcttggagaggtcctgaaggtctaattgaacacaatcgagctcaacgtcgttgtcaatattcagtgtctcattagaaggaaacatggtccctttcttgtaatgctgcttacagacttttaagccaattctattgtcttcattttctccataaccaagggtccccagggtaatgtcctttagctgatgatactgattaatagcaaaaaagatgctctcataggcatcctcttgagtatatacactgcagctgtagtcatcttcatctgtaccagaatatcctttcaaaaacaagtgcttaaaagcaacagtgttatcttctttgaaagcaaccaccagctggttacttaaaccaaaacgaacaagctgtgtggtgaccatgactatcttcaaaatctgcaaacccagtttccacggaatctggcgtctggctcggtatttttcacaagggctcatgaagtaaaacttcaggtcttcccttagacattcttctttcatctcagaatcacgatgtgccattgcatttctgacggttaacctgaaaacacctgatcctctctccggaatccttgcctggggaaaacgataaggctgccgggccatgcctcctccttcaaaactttccagggctctcgggattcggaacaggaaacaccgttcacggccgactcatttcgccctcgccgtaacgcgtccgccgaagttggagccctgcaaagcggggttcccttctcttaccctttctgccggccgcgtggtgcgcgcagaccccggcccgagagcaggcgccgcagtcgtggagtgcggcgggcagttctcgggcggctgaaaggcggctctgtgt

SEQ ID NO: 15815 - RNA, 6692 nt, Homo sapiens
  source 1..6692: mol_type = other RNA
gctgggattacaggcatgagccactgtgctcagctggcatttgttatataacagaccattccttgaaaatgccaacaaaacaaaacttttcaccaccctaaccagaaaaatgaacttttttttctaaattgccctatttctgtcagtgattccaatctcctaccaaagaaacatttactctgaaataattaagtccttaaaactctgtgttgaattgattactcttccccgctttcagtcttctaaggcctgtctgttcctatcacatgtttctccaatccacccttactactctactgtgatgtcaacacaaatttctgaattattaaagaaacttccaaggaagtctcttttactccaatctctttaccctccccagtcaaagctgcagtaaaacctgtactttaagaagaaggctttcaggtcatttctcccttgtgagattatacaaagtttggatgcaaaataaaaatctaaaccaagaaggttgtgataagttcctcctttatgcagcctcatcacatctcctccttgacagtattaatatgctgtgcttatcttctcctccaacaccaggcccatccctacatttttccctcatggaatttattctcctcacctgctctattcttctttctcttctctgtgtccaattaagccaatgttcaagggtcatttcagagtgtacttcaagaccaagtgccctggtagttctagtcctttctctgcactccgtatcggtaagaatcacagaatgaactatggtcttctaattgtttttatacacacttccctgtactccaactagatacaaacaccgtgccttacactaccagccacgtggctggaccaggcaaggtaaagttggtggccaagggagaaggtctacaaacgcaccccaaacaaggatcccacccatggctttgctgcatcagcaaaaactctgatgaactaaagtcctcctccaaaaagacctagaggaaatatccaaatgaacagatcacttaacaatatgtagattatttaacagtaaaacaggcgattgccagagtaaatattttccatacgctacacaagccttaaaacattgaagttaaagctgaaaacattgacattaaagttggtttctatggatgtcaactacaactctgacagcaccattaataattcacatttcttagtttcttttggaatccagtcaactcctttctctagtttcaagaacccctaactccaagcacaactgtctgtgcttcaggtttcaactgcaaatagctagtttgtcagtacatgtcacattcattttttaattttctgtttagttacttaccaggctacacacaatatctgtctcaacattaacattattcataaccattttacctccccctcctcttgtgaacatgagaattattttaacacaccaaagagttaaaacagagacccagtcaattttaggtgtttggtaacaccctgccattttgtacaagaagtggctgtgaaccagagtctatttcagtggccaaattccatagtagaagtgagcttaaaaatactcaaggtcctaatgtgcttccagtctagaaggaccacatttgtaaggcattcctttggatcttgagtgatcataagcccctggaaagcaggtactactctctctctgcttcttgtttgttcaaaacaaactttttgggcacctaccatggtctatgtgctgtgctggacactgggaatgtaaagaggaacaaactacagttccttccctccaagaacttggtctacaagaacctagcaatgttgggtgcacagtagatatttaatacgtattaaatgggtatttccataaagagtccccataggttctctgggcccacgatgagaactcaaccattcatttcacaaatgataagtttgcagttgggccaaaaacctttaatttcaatgaaaccataacctgcaatggcttatgtcagagaacaacataaatatttgctttaagagctggtgccaagaatctcatgcaaactttaggcaaaatgttttagctgaggggtacttggctaaaaccagagggcttggaaggaggaaaatgtaatgcagagtctgctgaactttgacccatggcatcagtgaagtccaacaacttttcaagtcttggtcttctcatttgtaaaatggggacaatgcaaggctatgatttattcctcacaggaaaaaaagtcctctggaaatgtaaaagccgcattagagtaatgtttaataattcaagatgaggtctggaagaacatcaacagtctctcaccctctgtgcccaggcattttgaaagggcactgtgccaaagtccattagtgctgggaatacacatcagcaggaagccttttgcatcttgactccctttccattgagcccctgaaatcagatgcctaacaggaagataggaagctgaagtgttatgggaccccagctatcagtcaaacggttttcctaatgtctcctttttagttgttttgttttaaagaaagaattagctttcacaatcaaggttgctgtgattctaaaaatcccacaaaaatgcccgcttggaatgcctagcttttcaaggcttcaggtaacctgaaagtcctctgattcagatactggcagaacctgaacatgctgacagcttggattaatttgggggaaaggatgcaaggggcaataaaatattctaacttcagattcaaagaggcagcaatatggtgaagaaaagcacaaagttccaaaaccagactgacgttctctcccccaactgacttgtacattcagtgaattaactcagctgtgtatttccccaatatatcagcctggtgagagatgccataaacagacctgcaggcaaccctacagacatcccttatccctcccctcctccaggggtataaaggaaagctaacattaagtgaaagacataagtctagagctgcaatgtccatagtggtagtcaccaggaatgtgtgaatagccagcatccaatagatagctagtccaaattgagacgtgctatgtggataaaatatccaccagatcaaaaagactagtatggaggaatgtaaaatatttcaatattttatactgaatacatgctgaaataatattttgggtatattaggcttaaaatatataattaaaaataatttcatctgtttttttatttcttcatgtagctactagaaaattttacagtataggcaaggctctcaattgtagcccaaactgtatttttcttggacagtgctggctcagagcatcccagtttcacctggatcctttgaaaggacaaattgaacatatggaaatgcagtcaggctcacaaaacaaataacctcattttccatgaggtgaccttgacaccattgaaagaatgaagccgattacatggctgtcctctcacagttgatctccaagtacaagactgtttcttgtcaggctaaatgctctcttgcaatgatctgttttagataataccaagaaaagctctacagggtatgggtcaaagcacaggtactggagtcaggccgacctgggtttgaatcccatctctgccactttctagctgggtaatctcaggaatattatttaatatattaaggtgcctattctctgtaacaggacaatcagatttcttcacagagaaggggagggaagggttaacacagcaagggagatgaagaatcttgggcaccatgcctaacagacagcacttgagaatggtagccatctagtaaaattctagcaatcttatctgagcaccttccagaataatgatgaggtaggggagacggggatggggtgcaaaggagatgggaccacttgtccacagaccttggagtcagtgaattaaagccgaatcctcaggaacggtatttattccacacagtgcaacactgccctctagtgacaaagaggtggaaaagctttcagagcatgaggcaagcaaggaagaaaaatacatttttccaggctctaagacagtaagttctccaaatcagagagatcatatcaaagaataattttttctcatgagtcacctttaaagcagtgacatggagtatgaagagcaatattatcaagatttactaccaacccagaggttgtcactttgttaattatataatatctcaaataggaaaaacagtaattctctctagacatattaaatgtgacacctaaaaagaagaaagtctgagtgttccaggttactcgacattattctggtaggacagcacggaggtttaagattcatgtataacagtttgtaaaccagatttgatcacagatttggttaatgcaactaacaaggtcaaaacttaaggctgaactggtatacaaacttggaaggaatacttaccatttttaacctcttttctccttgcagagcacctaagtgaggctaacagtaccctgggttgttgtggggagtaaataagaaagaacaccgaaatgcccagcagagtgtctaacacacaagcagtaagtgttagctgctgctatttttgttgtttctgttgttccaactgccacaggcccaaatggaggaaaagccataagataaaataactccttttacttttttgggttaaaaccaaggcttacctagtttcatttcctgatgcatctaccaatcaaatgtatcattttataacaagaacatcttagcacaactttgatgtccctgagattataatgctaactgaagtttggtaatagtttagaattcagatactgatctttaataaggcagaaagatgatgctgtaatcaaaaccgtctgcagagacaagacgtgtcaccatttctatcgtaaacctactatggtcgttttaggcagtctctgcccatcttcattcttctcaattaacttggatgaaaaacataatactttaaattggaaattttttataataattttcctcacttaattttcatttttaatatagtgatctcacgtccaaacatttcccatttgatgatcaccgggtaaccatgtgaccccttaagccagtcccagacaactataatacatgctttctagtattgtacagttcttgtttcaatatcctgtagtcacttctatatccttgtcatggtatggtcctaagacaatccagccacagaatgtgtaacccagataaatcataccagcacaagcacaaaaccgaagaacttttggcagtgaggcctgcattgttaaaatcagcacattatatgcctggaaataacccaggtatctgatgactccaacccaaaccaagagcgtagaggttccaagaaaaatgctgcagagatcatagtttgtgagattctttgctttgatttccatttttaatatggagccaatgattgtcattaggtcgctgataatcaccaggacataccagccgttgatgaactcccactggtcggtgtcacacacaggccgcttgtacttctccaggaagaaatttagaaatctcttccgtaaccttagagcaagaacaatggatcttgtacacagaataagagatgccaagcaaatcacaatgacaaatgcatcaaacaccaggacatactgagcatttttctgagtagatccaaatatgttcaagtctttacattcttcaattttggcatcactgtcaaaatagattttgattttgccactgtgagctttattgtcaaagataatcgtattctgaaagacataacagtctggtaactcacgggaatgaattgtctgtaggtcaatgcctttaagatgaaaggagatttcaacctgtaagagccgataaaattccagtctgaagaatgatgagttcttccagtccggaggcttcttggagaggtcctgaaggtctaattgaacacaatcgagctcaacgtcgttgtcaatattcagtgtctcattagaaggaaacatggtccctttcttgtaatgctgcttacagacttttaagccaattctattgtcttcattttctccataaccaagggtccccagggtaatgtcctttagctgatgatactgattaatagcaaaaaagatgctctcataggcatcctcttgagtatatacactgcagctgtagtcatcttcatctgtaccagaatatcctttcaaaaacaagtgcttaaaagcaacagtgttatcttctttgaaagcaaccaccagctggttacttaaaccaaaacgaacaagctgtgtggtgaccatgactatcttcaaaatctgcaaacccagtttccacggaatctggcgtctggctcggtatttttcacaagggctcatgaagtaaaacttcaggtcttcccttagacattcttctttcatctcagaatcacgatgtgccattgcatttctgacggttaacctgaaaacacctgatcctctctccggaatccttgcctggggaaaacgataaggctgccgggccatgcctcctccttcaaaactttccagggctctcgggattcggaacaggaaacaccgttcacggccgactcatttcgccctcgccgtaacgcgtccgccgaagttggagccctgcaaagcggggttcccttctcttaccctttctgccggccgcgtggtgcgcgcagaccccggcccgagagcaggcgccgcagtcgtggagtgcggcgggcagttctcgggcggctgaaaggcggctctgtgt

SEQ ID NO: 15816 - RNA, 3778 nt, Homo sapiens
  source 1..3778: mol_type = other RNA
gctgggattacaggcatgagccactgtgctcggcctgcaggttttaacaagaggagcatgaactatcattttgacacaaagacagcttaaaaaaaataataaagctggctggacgcggtggctcacacctgtaatcccagcactttgggaggctgaggtgggtggatcacaaggtcaggagatcaagaccatcctggacaacatggtgaaaccccgtctccactaaaaacacaaaattagccaggcatggtggcaggcgcctgtaatcccagctactcaggagggtgagccaggagaatcacttgaactcgggaggcagagcttgtagtgagcagagatcgcaccactgcactccagcctgggcaacagagtgagactccatctcaaaaaaaaaaaaaaaaaaaaaaaaaaaaagactatttgttgaatgttgaaaggaggagctaaaatcagttgaaattcggagtagaaggaaaactggagtgtctcattcacttcactctgatttgaatttttttttttttttgagacaagagtattgctctgtcacacaggctggagtacaatggtgcgatatcagctcactgcaatcttcgcctcctgggttcaagtgattctcctgcctcagcctcctgagtagctaggattacaggcatgcgccaccacacccagctaattcttgtattttttagtagaaatggggttttaccatgttggccaggctggtctcgaactcctgacctcaggtgatctgcccacctcgacctcccaaagtgctgggattacaggcgtgagccaccatgcccggcctgattttttttttttttttttttttgaggcagggtcttgctctgtcccccaggctggagtgcagtggcatactcatggctcactgcagcctccaattcctaaactccaatgatcttctcacctcagcctgccaagtagctaggattacagatgtgtgccgccatgctaatttttaaaaattttttgtatagatgggttctcactatgagcccaggctcatcttgaagttctgggctcaagcaatcctcttaccttggctttccaaagtactgggattacaggcgggagccaccatgccagccgtcactctcatttttgagcacaggaattgtgcccaaaggctaggataaggaattaaagatgcatgccaagaaatacccacaaacattaattataaaagggagactatactaatgtttgtgaaaagcttatactaacatagagcaatatttaagttataaagttaaatgaaaaagggtataaaactgtatgaacagtacaatctcaactatgtaaaaaccaaccaaaatctgccctaaaaaggctggaaggaaatagctcaaaatgttaatgtgattgtatttaagaagtgtatctaatagggatcttttttcttcctttttagttttctgtcttttccaaatgtttctctactggggagatttttttaaaaagctattagggaaggagtagaacaaaagtggaaaaaaaaatctattagttacaaaaaactgagtctgatagaagcattgaatttgagttaatgaatctaagtctagcctataagaatttgtacatttagaaaactatgaaacagtccaggctactccatgaatccattggtaggaccagaggctggaggtggaagtgccacctggtcctgcctgataaaaaatgctgaatcagccaggcacggtggcccacacacctgtaatcccaccattttgggaggctgaggtgggcggatcacctgaggtcaggagtttgaaaccagcctggccaacatgacgaaacactgtctctactaaaagtacaaaaattggccagcgtggtggcaggcgcctgtaatcccagctactcaggaggattacgtgaacccaggaggcagaggttgcagtgagccgagatggcgccactgcactccagcctgggtgacaagagtgagactccatctcaaaaaaacaaaacaaaacaaaacaacaacaacaaaaaaacccaaatcaatcaggaatgtcacatatttacaaaaaggaacagaaatactcacatttagcaaaaacttatttgtccattaatactataatcaaacatgcagattttctcgtattttctgtgcggatggcaagttacaaaaatgctattatcacaactgtagaatgtcaatcctagtttagaaacagtaataaaacagcacttcaacaagagtggaccgagaaagtgcacgacttagaaaattataaaaaatgcttcctacaaaaatgattccctttaagacatttgttcactgtacacattttaaggtcccctctcccaccccccaacaaaaatagaggcagaacctctaagcactttctaacaaagtgtcccctggtttgttcctctgacaaaccctgactgaaggctcatgatgtgcaggcactggggtctcaaagaggagaaagacttgtccctgcctcacggatgcctcagtcttcccaaagcaggaggcagacaagtcaccaaccgctacggatgtagaatggatgtattatacatccattaaaagcagatgccaatgccttcttaaaattaaacgatatgctgcaattcccactgaattacttatacaaacctccttacatacaagctgtcctgacttactaggaagcaaaaatgccaccaccttctcctgataaatacttctctaatgggcaggcattaaattacattttgtgatgtttgcccctaaacatcacaatgcctagtgaagtcagttaactttcttttaagcaatggtgcctattttactctgagaatgagacactttgaaactaaggaaggaaccagtcctgtatctagatcaagactcatcagtaccatcaaaagctgagatgaaacagtgtaagtttcaacagaaatcttcaatctcccatccgttgatgtgcaatgcgctcctgtgtcagccgctccaggtctttctgcacatttgggtggtcttccagatcttcgtagagcgacctgacgatgtccagtctcctgtaattctcaggcttgactaggctccggacaacctggaggcatcgctctttcagagtatacactagggttggctagttcctactccatcctgctctcttccttctccgggaagtgctccttaactgaaaccacacaaccgcaacccctccatctcccagcaggcaggtaagtcaatttcccacgccacacacggtcggctcttccggcgccaacatgaccctggcttgttcctgtctttgcatctgtcagtctccccaggaggaatgtgttctccacgagggcagggactacgcagaactggcccactggagtcatgaggactcggtagctgtggatgcggcggcccgtgccaggcggcagcgttgggtagggctgcggctcgccgtcgaagttgagccatacgggcagcacgacgcgcggactgcgattgcagaagatgacctgggagggctcgcgcgagttcaccgagcgcagcacgggccgcggccgcccggcctccatctcctcctcggcgcccagttcctccgggccggactcttccgggccggactcctcggcgcccgactcctccccgccgtcttcttcagggccgtactcttcgacgcctgcctcctccgcgcctacctcggcctcgtcccagttctccgccctccggggcattccctccgcgatccagaccacccgggccggacgccgcgggatccgcgggtcggacgcggggcggagctgc

SEQ ID NO: 15817 - RNA, 3519 nt, Homo sapiens
  source 1..3519: mol_type = other RNA
gctgggattacaggcatgagccactgtgctcggcctgcaggttttaacaagaggagcatgaactatcattttgacacaaagacagcttaaaaaaaataataaagctggctggacgcggtggctcacacctgtaatcccagcactttgggaggctgaggtgggtggatcacaaggtcaggagatcaagaccatcctggacaacatggtgaaaccccgtctccactaaaaacacaaaattagccaggcatggtggcaggcgcctgtaatcccagctactcaggagggtgagccaggagaatcacttgaactcgggaggcagagcttgtagtgagcagagatcgcaccactgcactccagcctgggcaacagagtgagactccatctcaaaaaaaaaaaaaaaaaaaaaaaaaaaaagactatttgttgaatgttgaaaggaggagctaaaatcagttgaaattcggagtagaaggaaaactggagtgtctcattcacttcactctgatttgaatttttttttttttttgagacaagagtattgctctgtcacacaggctggagtacaatggtgcgatatcagctcactgcaatcttcgcctcctgggttcaagtgattctcctgcctcagcctcctgagtagctaggattacaggcatgcgccaccacacccagctaattcttgtattttttagtagaaatggggttttaccatgttggccaggctggtctcgaactcctgacctcaggtgatctgcccacctcgacctcccaaagtgctgggattacaggcgtgagccaccatgcccggcctgattttttttttttttttttttttgaggcagggtcttgctctgtcccccaggctggagtgcagtggcatactcatggctcactgcagcctccaattcctaaactccaatgatcttctcacctcagcctgccaagtagctaggattacagatgtgtgccgccatgctaatttttaaaaattttttgtatagatgggttctcactatgagcccaggctcatcttgaagttctgggctcaagcaatcctcttaccttggctttccaaagtactgggattacaggcgggagccaccatgccagccgtcactctcatttttgagcacaggaattgtgcccaaaggctaggataaggaattaaagatgcatgccaagaaatacccacaaacattaattataaaagggagactatactaatgtttgtgaaaagcttatactaacatagagcaatatttaagttataaagttaaatgaaaaagggtataaaactgtatgaacagtacaatctcaactatgtaaaaaccaaccaaaatctgccctaaaaaggctggaaggaaatagctcaaaatgttaatgtgattgtatttaagaagtgtatctaatagggatcttttttcttcctttttagttttctgtcttttccaaatgtttctctactggggagatttttttaaaaagctattagggaaggagtagaacaaaagtggaaaaaaaaatctattagttacaaaaaactgagtctgatagaagcattgaatttgagttaatgaatctaagtctagcctataagaatttgtacatttagaaaactatgaaacagtccaggctactccatgaatccattggtaggaccagaggctggaggtggaagtgccacctggtcctgcctgataaaaaatgctgaatcagccaggcacggtggcccacacacctgtaatcccaccattttgggaggctgaggtgggcggatcacctgaggtcaggagtttgaaaccagcctggccaacatgacgaaacactgtctctactaaaagtacaaaaattggccagcgtggtggcaggcgcctgtaatcccagctactcaggaggattacgtgaacccaggaggcagaggttgcagtgagccgagatggcgccactgcactccagcctgggtgacaagagtgagactccatctcaaaaaaacaaaacaaaacaaaacaacaacaacaaaaaaacccaaatcaatcaggaatgtcacatatttacaaaaaggaacagaaatactcacatttagcaaaaacttatttgtccattaatactataatcaaacatgcagattttctcgtattttctgtgcggatggcaagttacaaaaatgctattatcacaactgtagaatgtcaatcctagtttagaaacagtaataaaacagcacttcaacaagagtggaccgagaaagtgcacgacttagaaaattataaaaaatgcttcctacaaaaatgattccctttaagacatttgttcactgtacacattttaaggtcccctctcccaccccccaacaaaaatagaggcagaacctctaagcactttctaacaaagtgtcccctggtttgttcctctgacaaaccctgactgaaggctcatgatgtgcaggcactggggtctcaaagaggagaaagacttgtccctgcctcacggatgcctcagtcttcccaaagcaggaggcagacaagtcaccaaccgctacggatgtagaatggatgtattatacatccattaaaagcagatgccaatgccttcttaaaattaaacgatatgctgcaattcccactgaattacttatacaaacctccttacatacaagctgtcctgacttactaggaagcaaaaatgccaccaccttctcctgataaatacttctctaatgggcaggcattaaattacattttgtgatgtttgcccctaaacatcacaatgcctagtgaagtcagttaactttcttttaagcaatggtgcctattttactctgagaatgagacactttgaaactaaggaaggaaccagtcctgtatctagatcaagactcatcagtaccatcaaaagctgagatgaaacagtgtaagtttcaacagaaatcttcaatctcccatccgttgatgtgcaatgcgctcctgtgtcagccgctccaggtctttctgcacatttgggtggtcttccagatcttcgtagagcgacctgacgatgtccagtctcctgtaattctcaggcttgactaggctccggacaacctggaggcatcgctctttcagagtatacactcggtagctgtggatgcggcggcccgtgccaggcggcagcgttgggtagggctgcggctcgccgtcgaagttgagccatacgggcagcacgacgcgcggactgcgattgcagaagatgacctgggagggctcgcgcgagttcaccgagcgcagcacgggccgcggccgcccggcctccatctcctcctcggcgcccagttcctccgggccggactcttccgggccggactcctcggcgcccgactcctccccgccgtcttcttcagggccgtactcttcgacgcctgcctcctccgcgcctacctcggcctcgtcccagttctccgccctccggggcattccctccgcgatccagaccacccgggccggacgccgcgggatccgcgggtcggacgcggggcggagctgc

SEQ ID NO: 15818 - RNA, 3642 nt, Homo sapiens
  source 1..3642: mol_type = other RNA
gctgggattacaggcatgagccactgtgctcggcctgcaggttttaacaagaggagcatgaactatcattttgacacaaagacagcttaaaaaaaataataaagctggctggacgcggtggctcacacctgtaatcccagcactttgggaggctgaggtgggtggatcacaaggtcaggagatcaagaccatcctggacaacatggtgaaaccccgtctccactaaaaacacaaaattagccaggcatggtggcaggcgcctgtaatcccagctactcaggagggtgagccaggagaatcacttgaactcgggaggcagagcttgtagtgagcagagatcgcaccactgcactccagcctgggcaacagagtgagactccatctcaaaaaaaaaaaaaaaaaaaaaaaaaaaaagactatttgttgaatgttgaaaggaggagctaaaatcagttgaaattcggagtagaaggaaaactggagtgtctcattcacttcactctgatttgaatttttttttttttttgagacaagagtattgctctgtcacacaggctggagtacaatggtgcgatatcagctcactgcaatcttcgcctcctgggttcaagtgattctcctgcctcagcctcctgagtagctaggattacaggcatgcgccaccacacccagctaattcttgtattttttagtagaaatggggttttaccatgttggccaggctggtctcgaactcctgacctcaggtgatctgcccacctcgacctcccaaagtgctgggattacaggcgtgagccaccatgcccggcctgattttttttttttttttttttttgaggcagggtcttgctctgtcccccaggctggagtgcagtggcatactcatggctcactgcagcctccaattcctaaactccaatgatcttctcacctcagcctgccaagtagctaggattacagatgtgtgccgccatgctaatttttaaaaattttttgtatagatgggttctcactatgagcccaggctcatcttgaagttctgggctcaagcaatcctcttaccttggctttccaaagtactgggattacaggcgggagccaccatgccagccgtcactctcatttttgagcacaggaattgtgcccaaaggctaggataaggaattaaagatgcatgccaagaaatacccacaaacattaattataaaagggagactatactaatgtttgtgaaaagcttatactaacatagagcaatatttaagttataaagttaaatgaaaaagggtataaaactgtatgaacagtacaatctcaactatgtaaaaaccaaccaaaatctgccctaaaaaggctggaaggaaatagctcaaaatgttaatgtgattgtatttaagaagtgtatctaatagggatcttttttcttcctttttagttttctgtcttttccaaatgtttctctactggggagatttttttaaaaagctattagggaaggagtagaacaaaagtggaaaaaaaaatctattagttacaaaaaactgagtctgatagaagcattgaatttgagttaatgaatctaagtctagcctataagaatttgtacatttagaaaactatgaaacagtccaggctactccatgaatccattggtaggaccagaggctggaggtggaagtgccacctggtcctgcctgataaaaaatgctgaatcagccaggcacggtggcccacacacctgtaatcccaccattttgggaggctgaggtgggcggatcacctgaggtcaggagtttgaaaccagcctggccaacatgacgaaacactgtctctactaaaagtacaaaaattggccagcgtggtggcaggcgcctgtaatcccagctactcaggaggattacgtgaacccaggaggcagaggttgcagtgagccgagatggcgccactgcactccagcctgggtgacaagagtgagactccatctcaaaaaaacaaaacaaaacaaaacaacaacaacaaaaaaacccaaatcaatcaggaatgtcacatatttacaaaaaggaacagaaatactcacatttagcaaaaacttatttgtccattaatactataatcaaacatgcagattttctcgtattttctgtgcggatggcaagttacaaaaatgctattatcacaactgtagaatgtcaatcctagtttagaaacagtaataaaacagcacttcaacaagagtggaccgagaaagtgcacgacttagaaaattataaaaaatgcttcctacaaaaatgattccctttaagacatttgttcactgtacacattttaaggtcccctctcccaccccccaacaaaaatagaggcagaacctctaagcactttctaacaaagtgtcccctggtttgttcctctgacaaaccctgactgaaggctcatgatgtgcaggcactggggtctcaaagaggagaaagacttgtccctgcctcacggatgcctcagtcttcccaaagcaggaggcagacaagtcaccaaccgctacggatgtagaatggatgtattatacatccattaaaagcagatgccaatgccttcttaaaattaaacgatatgctgcaattcccactgaattacttatacaaacctccttacatacaagctgtcctgacttactaggaagcaaaaatgccaccaccttctcctgataaatacttctctaatgggcaggcattaaattacattttgtgatgtttgcccctaaacatcacaatgcctagtgaagtcagttaactttcttttaagcaatggtgcctattttactctgagaatgagacactttgaaactaaggaaggaaccagtcctgtatctagatcaagactcatcagtaccatcaaaagctgagatgaaacagtgtaagtttcaacagaaatcttcaatctcccatccgttgatgtgcaatgcgctcctgtgtcagccgctccaggtctttctgcacatttgggtggtcttccagatcttcgtagagcgacctgacgatgtccagtctcctgtaattctcaggcttgactaggctccggacaacctggaggcatcgctctttcagagtatacactggcagtgtgatattggcaaaaataggctgtccgtcaacattgagagatggcacaaataattcagtttggttaaccagaagcccatcgtgtgtccctgcatctctgaagagccaaaggtgacctcggtagctgtggatgcggcggcccgtgccaggcggcagcgttgggtagggctgcggctcgccgtcgaagttgagccatacgggcagcacgacgcgcggactgcgattgcagaagatgacctgggagggctcgcgcgagttcaccgagcgcagcacgggccgcggccgcccggcctccatctcctcctcggcgcccagttcctccgggccggactcttccgggccggactcctcggcgcccgactcctccccgccgtcttcttcagggccgtactcttcgacgcctgcctcctccgcgcctacctcggcctcgtcccagttctccgccctccggggcattccctccgcgatccagaccacccgggccggacgccgcgggatccgcgggtcggacgcggggcggagctgc

SEQ ID NO: 15819 - RNA, 3114 nt, Homo sapiens
  source 1..3114: mol_type = other RNA
gctgggattacaggcatgagccactgtgcttggccaaatcctttttaacaaacaaacaaaaaaaaaacttcttgcttttgttgcctcctaaaacatatcaaagtcttacagtctgaaaagtacttttccgatacaagacaatttaatattttcatgccattttctcattgtaaacacacatcaatataaaattgtcatgaaaactacatttgaaattcaaatggtgatggttttaaccccaaattaacatttttagaggaaataatgtttggtggaaatgttcattaaacatcattacaaatttaatgaaaaagcatgcatttgtacaagataggataccccaggtatattcagtcccatgattttttttgaatgtcatctaaatcaaacatgaaatatgctttatgtacaggcatgaccattacttcatgtgacttactgaattctgtctagtctttggtcccatagaaattattatctacatcaacctcgctgattttttttcatctctctttttagtaggttccattcaaggcaaaatgaaaacttttgtcaagtactaatgtaaaatttcaaaatccagttttattctcaaaaacttatttgcatcttccactgttaagacagtggtctctgactctgttttgttaactctataaagccagtttcacaggataaatttgaatcaacagtgcctactactgcatcccaggtcaccagtacaacactgaattgactcctgaggtaaaccgactgtatctcataatgacaggcttccaaagctctgtgcgctagctacaattggaagcaaatgccacctgtgcaaacagacttcagaaagccttctttccacttaatagatatgtctatgtaaatggccaaaaaattcatcattgtgtgtccatgatcatattttaaaatacatagttcacaatattacttctcttaaaattaaagaattaaagctcaaatttttttttctaaataaattggctttaaaatgtagactgcaaatattcctgaccatattgatgggccagttcacaatctatgaagagttgaacatatatatggaatatatatgttccctttcatgtctgaagaggaataaaactgtacagcattgtcttttgtttctgaaacataatttagaactaaaataaaattgaaaaataattctcactagacctaggaatttcctaaatggatcaaagtactttttaacacacgtgggatttaattaaaacgacttgaattcttgttaagataacaagttgcagcatcgcttactagctcattctgtttgtttctgtgtctggtccacttatatggaaactcaaccataaggatactctatcttttatcacacatgagtacaattggttgatggtggggtgtctattcgacttttactttctttagtatcactcaggtgtgaatctttgcgaatgtgacacttgaacacttgtttataggccttcctgaaattttcagagagaaatgcataaatgataggattcacggaggaattgctgtacgccaggcagtgggcggtgattctgaagaggaaggaagccggcgtcagcgggaaaactccaaactcagcccagagatggatgatgtggtgcggcagccaggagattccaaacaccacaaccaccaccagaactgtctgtgcagtctttttcttggatgcttcagacttctttgacatgttcttcaactttttatgcaagtgattaaggaccttggcatagcagaagcagatgagcaggagcggcagcaggtagccgaagacgaaggtgcacaccacgtaggccttcttgtggcgagggtcgggccactgctcccagcagaaggtctggttgctggcgcgcgggtggaagaggccctggtggtaggccacgggcgaggccatggcaatggacagcgcccagatgcagcccacgcccagcagcgcgttgcgggacaccctgagggaggaggagcgccgcgagtgcacgatggccacgtagcggtccacggacatcgcggccagggtgaagatgctcaccagcatggacacggtgaagaagtagtggatgaacttgcagatgaaggcgcccagcacccaggtgggcagcgcgtacacggtggcctggaaggggatgcagaagagcaggtaggccaggtcggcgatgctcaggttgaggatgaacaggttggtggtgctccgcggcttgcccggcttgctgcgcgccagcacggtgatcactaggctgttgcccagcacacccagcgcgaagatcaggccgaacaccaccagcgtgacgaagttctccacgccgatgccgaacagcggcccgggctccggggcggggggctccggccagctcgcgttgccctcgctgaggttcccgaccgccagctccatggcccgcggggctgtcccggcgagcggcggggcgcgcggggagggagggcgggatagtaggcgccgggggtggccaggggtcccggcgcaaagcacggagagtgcgagtttaggagtctgagcttcccccgaggcgcgagccagcgggagcggggatccggtggccgtgcctggtggcaccgtctttgcgccgggaccttctgagagagggtgggttcgggagcccggagctggaccttctcgggaagggacggtgatctcgagagcactggggtccccttcccgggcgcctccgcccgctgcgcgaccacggagcctgggaagagggatccgccggctgcagccgcgcaggtggaaagacccttctctccgccttaccgctccagatcttcgccggcggttttccctggctcccggaggggctgcgtgctgcacctgttgctcggagccgctccttcccgcggcgcttccccgcactgcccagcgcgcagcagtgcactgtgcggctcctgcagagaaggctccccgcgcatcccgcgcgcccagcgccacctccccagtgggctggcgcctccgactccctcccggcttttccagggattccgagtcgtccacagggcgagagctcttttgggaggcttcctggtggtggatagagtcgggtgccaggggcttctctgctgcaactgagaggcgaaaac

SEQ ID NO: 15820 - RNA, 3863 nt, Homo sapiens
  source 1..3863: mol_type = other RNA
gctgggattacaggcatgagccactgtgcttggcctcagtgctggcctcagttttggggttctaggaacagagctggtgcaaatgttcttaattgtttcttttggtgtgtgttggggggaatggcgggggttgggtaagaacttctccagggcatttgcaaggccattgggaaagtacattgtcaacttcagtagataatgccaaaattttaaaaagtggttataaccattcgcacacccactagtagtttgagcattcccctcactccacttcttcaccaacacctgcaattatcagcttttttttttttgtagatggatctgtgtgaaattgtaactcactgtggttttagttttcatttccctggttatgcatgctgccttttttttacttaaaatatgtcttggtgactgttccgtatcagagcagtgaggacttcctcctcctttcttggctggaaagtgttccatcgtcatatggaaatcttgtggtcgatttaacccgttccctattgatagacgctgtgtgggctccagccttttgcagtcgactctgcgatgcataacttcgtgtatagatagcagtctgcagctgcacgtgggggtgtgtgcatgtaggtttttcacaggaacctcctgaaatgctcccccaactctgctttgatgtggtatcctgcaggcatagggagtgccatggactggtgcctggggaattgcatgggaaaggaaaagatgaattgcatgtgccctccaggaagtttggaagctggtctggagagtgtgaagccagggctggctaaacatctacagcaaccatttctagctaagagctttaaactcattagtctcaatctcccaacagtccaggtgggttggaggcattatgtaattgtcatgcccctttcctgcacagattgagccccagagaggttgagtagcttgggcaaggtcacacagctgggaagcagtggagctggaattcacaagtccgtctgattctagagcccatgcacagcgtttctttctctcccttcctcttccacctcctttttctcctcctcctccttcctctctctctctcttagataattgcatttacatggtctcaaaatcaaagggtacaaaaggatatacagtgataatcctcttcctactatttcccagttttccttcctagagaaaagtaagggtactagtttcttgcaactagctttagaatattcaattcatatataaatgagtatattccatagatattcttccccattttttagacaaaaaaaatggtggcatcctatatgtactgtttggcactgagggttttgtttttttttttaacttagtatttcttgatagtctttccctgtcagttcataaaaagcctttccttattctgctttattatctgcatactcaactcatcctctatttggtggatgtagagggggctcccgaccttatgcagttacaacccattctgtgtgagcatccctgacctcaggtgcagaaggcatgagcagcacatctgtcagataacacatctgtcagatgacaccctagaaggggagatgctgaacacacttggtgccattcgttagcttctcctcaaatctgctcacagacttaaccataacgatacttctttcttctataatctggctgctccagcatgttcctctgacagcactttctcccacagactctgttgccaaacttgggtctgcccaccaggtgcagcaaagccaagcactgacattgggatttgcagcaagagaaagtgaggcatttactgcagggtgccaagcaaggagaatcgggcagctcatgcttaagccccgaactccagggtggctcacaggtaagggtttttaaaggcagggaggcagaggttacaggcaaagtcataaatcaatacatggaaactgtgcattggtttgacctaaaagggtgggacatctcgaagcggggcccgcaggtcataggtggattcaaagatcctctgatttgtgattggttaaggaggcaaagctttgtctaaaaacctggggtcagcagaaaggaatgttgagctctggcctgtgggtgtgacttcctccaggcccctcaggaagaaatgttgaacaaagaatggtggtctgagttcagtcctcggctcccaactgaagtctctgtgccagtggatggcattttccatttgctgggggcctgggtttaattgcacaattcgagctccgtccttttgccacggctttgagctctgttgaaacaagatcctcccaggtgtttctcagtcttctaatgctcaggcctgcttttcatgacataaacagctctgtccctttctgtagttctaattacaaaaacaaaaggttcttcccacacgtaaaattacatagtactcttaaatatgtcttcttgaacgccatcgccccatcccagactcaggaccagcctccccgcgctcactgctgtcactgctttccgcactccctgcggattttaggattttagctcccatctcgcgtcctctctccagctcctcctgccccctgcctggtggtttcaccatccacttaccagcccgccgatggtgccctggcctcccagttctttgacctcctctccccagtgatcttccagggctcggcactcagtttcctggtcaagcttgagccctccagagaagccactgtcaaacctctttccggctcgtgccttggagccatcgcccctcagggccccacagactactgacctcacccgctttcaaatccctactccctcctttcccagcctaaattccagggttagttattctagtccctaccttttctatacccttccctccacactccaagttggactgtacttgcttggcaaaaccccaacccagttagatccagttctccgccaactctgcctgctctactgtgtgtcttacttgcttattttattacctctgactccctccaccagcatgttgaccccacggggacaggggctatgtccctgctgctctgccctagcagccaaagaatatctggtacatagtaagtgcatattcattaaagtgtatagtcgatgaatgaatttttctaggtgtggagaaagatctgagagcaggtttaccatagtatctggggaaaaagcagaggggggacgttgtgttgtgtccaagggggctagaggagggtcaaggaggaaggcataaggaggccaagcccaggggctcctccagtttgcccagagaatgccaccattctttcctaattagctccttttggtctgggagaagctcttagaagagtatttcattctcgagccctaatcacaggattctgaacccttactaaactgttgcttcctgcagtcttggttactcagggctcccgagccaacgtttggatggctgtgattatctgggatgtctcaggaatgacctaaccacttacctcttccaagttctgaattttacaacaggaaattgaggcccagagaacagaaggacacatgggtgctgctggtagagcccgaactggaacccagatctgcctccagtcccgggctcatctgccaccgtgtaccatgccctctctctgttgtcacatgcagtcacttgcccgattgtccacaccctgcaaaacttgcttcctgagcgacaggacagttctcagggccctgcatgtagcacctcatctactcctccaacagccctctgagggaggctctgttattattacttctattttattgagacacaaggaaattgcgtaaccacacacattattaggaagtgacacagcctaaattcaaacactgcttcactcgggctcgtgcttataaccttacctaggtgtcttaaa

SEQ ID NO: 15821 - RNA, 2761 nt, Homo sapiens
  source 1..2761: mol_type = other RNA
gctgggattacaggcatgagccactgtgcttggcctcagtgctggcctcagttttggggttctaggaacagagctggtgcaaatgttcttaattgtttcttttggtgtgtgttggggggaatggcgggggttgggtaagaacttctccagggcatttgcaaggccattgggaaagtacattgtcaacttcagtagataatgccaaaattttaaaaagtggttataaccattcgcacacccactagtagtttgagcattcccctcactccacttcttcaccaacacctgcaattatcagcttttttttttttgtagatggatctgtgtgaaattgtaactcactgtggttttagttttcatttccctggttatgcatgctgccttttttttacttaaaatatgtcttggtgactgttccgtatcagagcagtgaggacttcctcctcctttcttggctggaaagtgttccatcgtcatatggaaatcttgtggtcgatttaacccgttccctattgatagacgctgtgtgggctccagccttttgcagtcgactctgcgatgcataacttcgtgtatagatagcagtctgcagctgcacgtgggggtgtgtgcatgtaggtttttcacaggaacctcctgaaatgctcccccaactctgctttgatgtggtatcctgcaggcatagggagtgccatggactggtgcctggggaattgcatgggaaaggaaaagatgaattgcatgtgccctccaggaagtttggaagctggtctggagagtgtgaagccagggctggctaaacatctacagcaaccatttctagctaagagctttaaactcattagtctcaatctcccaacagtccaggtgggttggaggcattatgtaattgtcatgcccctttcctgcacagattgagccccagagaggttgagtagcttgggcaaggtcacacagctgggaagcagtggagctggaattcacaagtccgtctgattctagagcccatgcacagcgtttctttctctcccttcctcttccacctcctttttctcctcctcctccttcctctctctctctcttagataattgcatttacatggtctcaaaatcaaagggtacaaaaggatatacagtgataatcctcttcctactatttcccagttttccttcctagagaaaagtaagggtactagtttcttgcaactagctttagaatattcaattcatatataaatgagtatattccatagatattcttccccattttttagacaaaaaaaatggtggcatcctatatgtactgtttggcactgagggttttgtttttttttttaacttagtatttcttgatagtctttccctgtcagttcataaaaagcctttccttattctgctttattatctgcatactcaactcatcctctatttggtggatgtagagggggctcccgaccttatgcagttacaacccattctgtgtgagcatccctgacctcaggtgcagaaggcatgagcagcacatctgtcagataacacatctgtcagatgacaccctagaaggggagatgctgaacacacttggtgccattcgttagcttctcctcaaatctgctcacagacttaaccataacgatacttctttcttctataatctggctgctccagcatgttcctctgacagcactttctcccacagactctgttgccaaacttgggtctgcccaccaggtgcagcaaagccaagcactgacattgggatttgcagcaagagaaagtgaggcatttactgcagggtgccaagcaaggagaatcgggcagctcatgcttaagccccgaactccagggtggctcacaggtaagggtttttaaaggcagggaggcagaggttacaggcaaagtcataaatcaatacatggaaactgtgcattggtttgacctaaaagggtgggacatctcgaagcggggcccgcaggtcataggtggattcaaagatcctctgatttgtgattggttaaggaggcaaagctttgtctaaaaacctggggtcagcagaaaggaatgttgagctctggcctgtgggtgtgacttcctccaggcccctcaggaagaaatgttgaacaaagaatggtggtctgagttcagtcctcggctcccaactgaagtctctgtgccagtggatggcattttccatttgctgggggcctgggtttaattgcacaattcgagctccgtccttttgccacggctttgagctctgttgaaacaagatcctcccaggtgtttctcagtcttctaatgctcaggcctgcttttcatgacataaacagctctgtccctttctgtagttctcttccaagttctgaattttacaacaggaaattgaggcccagagaacagaaggacacatgggtgctgctggtagagcccgaactggaacccagatctgcctccagtcccgggctcatctgccaccgtgtaccatgccctctctctgttgtcacatgcagtcacttgcccgattgtccacaccctgcaaaacttgcttcctgagcgacaggacagttctcagggccctgcatgtagcacctcatctactcctccaacagccctctgagggaggctctgttattattacttctattttattgagacacaaggaaattgcgtaaccacacacattattaggaagtgacacagcctaaattcaaacactgcttcactcgggctcgtgcttataaccttacctaggtgtcttaaa

SEQ ID NO: 15822 - RNA, 2526 nt, Homo sapiens
  source 1..2526: mol_type = other RNA
gctgggattacaggcatgagccactgtgcttggcctcagtgctggcctcagttttggggttctaggaacagagctggtgcaaatgttcttaattgtttcttttggtgtgtgttggggggaatggcgggggttgggtaagaacttctccagggcatttgcaaggccattgggaaagtacattgtcaacttcagtagataatgccaaaattttaaaaagtggttataaccattcgcacacccactagtagtttgagcattcccctcactccacttcttcaccaacacctgcaattatcagcttttttttttttgtagatggatctgtgtgaaattgtaactcactgtggttttagttttcatttccctggttatgcatgctgccttttttttacttaaaatatgtcttggtgactgttccgtatcagagcagtgaggacttcctcctcctttcttggctggaaagtgttccatcgtcatatggaaatcttgtggtcgatttaacccgttccctattgatagacgctgtgtgggctccagccttttgcagtcgactctgcgatgcataacttcgtgtatagatagcagtctgcagctgcacgtgggggtgtgtgcatgtaggtttttcacaggaacctcctgaaatgctcccccaactctgctttgatgtggtatcctgcaggcatagggagtgccatggactggtgcctggggtcagcagaaaggaatgttgagctctggcctgtgggtgtgacttcctccaggcccctcaggaagaaatgttgaacaaagaatggtggtctgagttcagtcctcggctcccaactgaagtctctgtgccagtggatggcattttccatttgctgggggcctgggtttaattgcacaattcgagctccgtccttttgccacggctttgagctctgttgaaacaagatcctcccaggtgtttctcagtcttctaatgctcaggcctgcttttcatgacataaacagctctgtccctttctgtagttctaattacaaaaacaaaaggttcttcccacacgtaaaattacatagtactcttaaatatgtcttcttgaacgccatcgccccatcccagactcaggaccagcctccccgcgctcactgctgtcactgctttccgcactccctgcggattttaggattttagctcccatctcgcgtcctctctccagctcctcctgccccctgcctggtggtttcaccatccacttaccagcccgccgatggtgccctggcctcccagttctttgacctcctctccccagtgatcttccagggctcggcactcagtttcctggtcaagcttgagccctccagagaagccactgtcaaacctctttccggctcgtgccttggagccatcgcccctcagggccccacagactactgacctcacccgctttcaaatccctactccctcctttcccagcctaaattccagggttagttattctagtccctaccttttctatacccttccctccacactccaagttggactgtacttgcttggcaaaaccccaacccagttagatccagttctccgccaactctgcctgctctactgtgtgtcttacttgcttattttattacctctgactccctccaccagcatgttgaccccacggggacaggggctatgtccctgctgctctgccctagcagccaaagaatatctggtacatagtaagtgcatattcattaaagtgtatagtcgatgaatgaatttttctaggtgtggagaaagatctgagagcaggtttaccatagtatctggggaaaaagcagaggggggacgttgtgttgtgtccaagggggctagaggagggtcaaggaggaaggcataaggaggccaagcccaggggctcctccagtttgcccagagaatgccaccattctttcctaattagctccttttggtctgggagaagctcttagaagagtatttcattctcgagccctaatcacaggattctgaacccttactaaactgttgcttcctgcagtcttggttactcagggctcccgagccaacgtttggatggctgtgattatctgggatgtctcaggaatgacctaaccacttacctcttccaagttctgaattttacaacaggaaattgaggcccagagaacagaaggacacatgggtgctgctggtagagcccgaactggaacccagatctgcctccagtcccgggctcatctgccaccgtgtaccatgccctctctctgttgtcacatgcagtcacttgcccgattgtccacaccctgcaaaacttgcttcctgagcgacaggacagttctcagggccctgcatgtagcacctcatctactcctccaacagccctctgagggaggctctgttattattacttctattttattgagacacaaggaaattgcgtaaccacacacattattaggaagtgacacagcctaaattcaaacactgcttcactcgggctcgtgcttataaccttacctaggtgtcttaaa

SEQ ID NO: 15823 - RNA, 2465 nt, Homo sapiens
  source 1..2465: mol_type = other RNA
gctgggattacaggcatgagccactgtgcttggcctcagtgctggcctcagttttggggttctaggaacagagctggtgcaaatgttcttaattgtttcttttggtgtgtgttggggggaatggcgggggttgggtaagaacttctccagggcatttgcaaggccattgggaaagtacattgtcaacttcagtagataatgccaaaattttaaaaagtggttataaccattcgcacacccactagtagtttgagcattcccctcactccacttcttcaccaacacctgcaattatcagcttttttttttttgtagatggatctgtgtgaaattgtaactcactgtggttttagttttcatttccctggttatgcatgctgccttttttttacttaaaatatgtcttggtgactgttccgtatcagagcagtgaggacttcctcctcctttcttggctggaaagtgttccatcgtcatatggaaatcttgtggtcgatttaacccgttccctattgatagacgctgtgtgggctccagccttttgcagtcgactctgcgatgcataacttcgtgtatagatagcagtctgcagctgcacgtgggggtgtgtgcatgtaggtttttcacaggaacctcctgaaatgctggggtcagcagaaaggaatgttgagctctggcctgtgggtgtgacttcctccaggcccctcaggaagaaatgttgaacaaagaatggtggtctgagttcagtcctcggctcccaactgaagtctctgtgccagtggatggcattttccatttgctgggggcctgggtttaattgcacaattcgagctccgtccttttgccacggctttgagctctgttgaaacaagatcctcccaggtgtttctcagtcttctaatgctcaggcctgcttttcatgacataaacagctctgtccctttctgtagttctaattacaaaaacaaaaggttcttcccacacgtaaaattacatagtactcttaaatatgtcttcttgaacgccatcgccccatcccagactcaggaccagcctccccgcgctcactgctgtcactgctttccgcactccctgcggattttaggattttagctcccatctcgcgtcctctctccagctcctcctgccccctgcctggtggtttcaccatccacttaccagcccgccgatggtgccctggcctcccagttctttgacctcctctccccagtgatcttccagggctcggcactcagtttcctggtcaagcttgagccctccagagaagccactgtcaaacctctttccggctcgtgccttggagccatcgcccctcagggccccacagactactgacctcacccgctttcaaatccctactccctcctttcccagcctaaattccagggttagttattctagtccctaccttttctatacccttccctccacactccaagttggactgtacttgcttggcaaaaccccaacccagttagatccagttctccgccaactctgcctgctctactgtgtgtcttacttgcttattttattacctctgactccctccaccagcatgttgaccccacggggacaggggctatgtccctgctgctctgccctagcagccaaagaatatctggtacatagtaagtgcatattcattaaagtgtatagtcgatgaatgaatttttctaggtgtggagaaagatctgagagcaggtttaccatagtatctggggaaaaagcagaggggggacgttgtgttgtgtccaagggggctagaggagggtcaaggaggaaggcataaggaggccaagcccaggggctcctccagtttgcccagagaatgccaccattctttcctaattagctccttttggtctgggagaagctcttagaagagtatttcattctcgagccctaatcacaggattctgaacccttactaaactgttgcttcctgcagtcttggttactcagggctcccgagccaacgtttggatggctgtgattatctgggatgtctcaggaatgacctaaccacttacctcttccaagttctgaattttacaacaggaaattgaggcccagagaacagaaggacacatgggtgctgctggtagagcccgaactggaacccagatctgcctccagtcccgggctcatctgccaccgtgtaccatgccctctctctgttgtcacatgcagtcacttgcccgattgtccacaccctgcaaaacttgcttcctgagcgacaggacagttctcagggccctgcatgtagcacctcatctactcctccaacagccctctgagggaggctctgttattattacttctattttattgagacacaaggaaattgcgtaaccacacacattattaggaagtgacacagcctaaattcaaacactgcttcactcgggctcgtgcttataaccttacctaggtgtcttaaa

SEQ ID NO: 15824 - RNA, 1479 nt, Homo sapiens
  source 1..1479: mol_type = other RNA
gctgggattacaggcatgagccactgtgtccagcctgctttttcaaaattattaccacactggttcacactgaaggtaaaagcaatagctagaatctcttattaacaacacattttgacttcaagttcagacaaagctgttggttacaagttcagctgaatttttgtcaaatttaagaagtctgtaggacaacacaaaaccatccctggtaatatatttgcagtctggtcttcaaaagtgtggcctggagttatgacaccaacttgtatttggccaattaaggaagaggccaaactgcattcttcttagaaggtctattcagttgataagtggcacttaactgatgttttttttcatataacctttgcattgattatgccccaagagataagggacagatggtaattcagatgagaacctctgaaaagatttatcagttttctgtcccgttccagccagattttttggaaaaccttggggaaagactgaaattccccaccaatctgagactgtatgcgagtttttacaacattaattggaaaaaacaggaatcccaacatggcacccaatagacctccaccgataaaatcattgaccaaatgagaattgtgagtcgtcgcggtaggcagatgctccttaacgtgacctcgaaggccgaaaaaaaaaagacattgctgagtccattctggaaaagaatgggcaccaaacctcgataaaactctccaattccatgacatttcagtgccttgaaagcctgataaatgttggcaaatttgtcatggtgcttgtggtcttgaagcaatgtctgaagtgaaaattgcttccgttgtccctgcaagcactgctgccacgccacaggttgcaaactctggagcactgacatgcttgtggagaaggtaggataaatcctcatacagaccaaacgtaagtgcaagtgtagttgtcttctgcatcaatcggggaaagattccccgatacaagtttcgaaatccatccgttctcaactgaagtattgcatcccccgttttgatgccatacagctgttgtggaaagaggaccttctgaatgggaaatgtgattgcgacgttgttgaaggctgcacagcagccacacaagtaatgcttcatttcactaaatctgtaatatgaggtgacatatcttgtttcgaagatgttagtattggtggtctctttccatgagcttctgaatccatcatgttgcttaagttcttcttttttcatgaaggactttttctttttttttttttaaacctgtaacaccatccaagcctggagtttaacagaatgatagctttttgataatattcccaatttcttccattgttattgttctgttaggttctctcttctggagtcaattttgataactggatttccgttctccaggcgtccatttccccagtcgcaggagaaagagccgggaaccgaagagactcaactgattccgcgcgcgccgcct

SEQ ID NO: 15825 - RNA, 1624 nt, Homo sapiens
  source 1..1624: mol_type = other RNA
gctgggattacaggcatgagccactgtgtccagcctgctttttcaaaattattaccacactggttcacactgaaggtaaaagcaatagctagaatctcttattaacaacacattttgacttcaagttcagacaaagctgttggttacaagttcagctgaatttttgtcaaatttaagaagtctgtaggacaacacaaaaccatccctggtaatatatttgcagtctggtcttcaaaagtgtggcctggagttatgacaccaacttgtatttggccaattaaggaagaggccaaactgcattcttcttagaaggtctattcagttgataagtggcacttaactgatgttttttttcatataacctttgcattgattatgccccaagagataagggacagatggtaattcagatgagaacctctgaaaagatttatcagttttctgtcccgttccagccagattttttggaaaaccttggggaaagactgaaattccccaccaatctgagactgtatgcgagtttttacaacattaattggaaaaaacaggaatcccaacatggcacccaatagacctccaccgataaaatcattgaccaaatgagaattgtgagtcgtcgcggtaggcagatgctccttaacgtgacctcgaaggccgaaaaaaaaaagacattgctgagtccattctggaaaagaatgggcaccaaacctcgataaaactctccaattccatgacatttcagtgccttgaaagcctgataaatgttggcaaatttgtcatggtgcttgtggtcttgaagcaatgtctgaagtgaaaattgcttccgttgtccctgcaagcactgctgccacgccacaggttgcaaactctggagcactgacatgcttgtggagaaggtaggataaatcctcatacagaccaaacgtaagtgcaagtgtagttgtcttctgcatcaatcggggaaagattccccgatacaagtttcgaaatccatccgttctcaactgaagtattgcatcccccgttttgatgccatacagctgttgtggaaagaggaccttctgaatgggaaatgtgattgcgacgttgttgaaggctgcacagcagccacacaagtaatgcttcatttcactaaatctgtaatatgaggtgacatatcttgtttcgaagatgttagtattggtggtctctttccatgagcttctgaatccatcatgttgcttaagttcttcttttttcatgaaggactttttctttttttttttttaaacctgtaacaccatccaagcctggagtttaacagaatgatagctttttgataatattcccaatttcttccattgttattgttctgttaggttctctcttctggagtcaattttgataactggatttccgttctccaggcgtccatttccccagtctgtgaaaagcggggagggggttggacaagatcactaaaccctgttccgtctttgacactccacagtcagcggtcccgaggtgaggaggccagaaatcccagtctcccgggaggcaggggcccttgcgcggtgccagctctgctccctccggagctcaggcagagccaggctcctacccgcccctgcggttcctgcgcacc

SEQ ID NO: 15826 - RNA, 4179 nt, Homo sapiens
  source 1..4179: mol_type = other RNA
gctgggattacaggcatgagccactgtgtctagctgactggagaagcttttaaaatagactgacatacatctcccgctgcacaacagctaagtcagaatcttggcggtagggagtatggattctgtctttccagttctctacaataacctgaggtgtgatgacatgagccattttgcacaccactggatacccgaaaatgctacaaacacctattcagcccctcattatgcctgtctgtcacagggaggctggaaacctatagctaagtaaggagactgtgtgtgctgttcatcaagggaacgtgtgacttccacacatgctggacaccagagatgaggcccaagctggtgaagggcccacatggaggtaaggatcacaggcttgattgggagggaaagacaagtggaaaatggcaagaagaggaggaactgggagaagcaaaacaaggcgaagataaatttaataattttctttaaataaatttgttatgctaaaaaaaaaacctctagtcattttctagagacttctttttgccttagggattctttatagttcctctccatgtaacatattgggtaatacttgtggttctgaaataaaatgcaagcaggggggtgtacacaaaaaccttaccactgaatcaagggaccagctgtgcagacattatgtaacagtaatattctatagttctgaacatggcacttgtgaatcaataattttagaatattttagaaaggacatttaaaaaaatcacataggaaacaaagttaaaatttagaaaaaagtagaatattttatcccatcttctaagcacctcaagcctaaacaaaacacacagaatgaaattttaatgatgcctgttaagcctatttgaaaacaaattctatctggcccccataaacggatgttcaggtgttcaggcaatcaactccttggttctccaatctgaaatgttcaaaggaaggaggtagaacttgggcaagtttaaagcatgtagctctgttgaatcacttctaaccaccccgcccccagctgatgaccaatttttacactgaccacagctgaaaatgtaaatgcaaataaaaagcttgagatgttattggacgaggtgtattaaaataaaatcaaaaatagaaatattaggtatatacacaacagcataagtgaaacacatcatgtgatacagaagtttccattcaaagcttacaggagaaaaatttagtgaacagaaccgcttgaacctcctgccaccgtggcttattagagccttgtagtcacttatgttccttcatatccttgggtataaatagtctcatacacatgctacacaatttagaaaagattgctgaatcataaaaatagccccgaatgtggcactttagctttctagagtacaactaaaattaatacttgatctttaacataatgttcaaatatttgaagcaacaaaggaaactcttatgttttagaaggccctataaggttcttcagagattagaatcttagttcttccaaactacattgtcaaaacaaatctggatataggaaattgtggaaatgaaaaagctggactcttaaaaatattccttctaaacacagagcagtttctgaggctcttctccctttcctgggaggtccaggtgagcccggtgccttcgggtgagcagacagggcagctgtgcgtgctcacgggctcctcctgctggaagagagagagatgtgcacgccactcctatggcatgtctagcaggtctgagcagtgttcatagaagaaaaatgttttaacagtctcagattttgggaggtagggggaaaaaaatcattgaaatctgggaaagacatttttaagctgctgacttcacctgcaaaatctaacaggttggattagtttttttttttttttaaacaagtaagccaaagcacaaagaaatgtcatgctatgtatatatccggttattttagctttataaatgagtttagttctgcaattattggggattcattgcaatggtctctgaaactttgagtcctatgtccatttgtaaacatagagctagttgggtgcatttttggagagaatagatgttttcttctcaaacggctgcactcagatgttgtcaagcagagcaagattaccagctgctgaggacaagtccaagttgcaactgagtggagaatccatctaagagtacagaatactttcccatttagagggtgttcttcctgagtaatttagcctctatttcaggatccaggcacggcagatgatccccgcacatgaaatcataagtgcaaccagtgatggttacttttcctctctaaatgaggcagccacccctgccaaatggacgggtctccctgtgctctaaggctgctgctggtattgcccttccgtggctgtgtagaaatcatccaggacgctctgtaagtagtcaaacgttggtctctcttctgccttttctttccagcacattttcataatgtcatagagctcatctgggcagttctccacacggggcatcctgtagccctgggacagggcggtcatcacgtcggcattagttctccctgggtagggaattttcccataggtgacaatttcgtataggaggattccaaaggaccacacatcagacttaatagtgaaacatccaaagttgattgcttctggagccgtccacttaatagggaacttagcaccttcccttgctgtgtactcattatcttcaattactctagcaaggccaaaatctgcaattttgcacatgagtgactcggagaccagaacattagctgctcgcaggtcccggtgaatgtagttcttccgctcgatgtatgccattccctctgcaatctgagcagaaaagtcaatgagctttggaagcagcactttgccaccttcatcgctcttcaggaaatccagcaaactgcccttggccatgtactcggtgatgatgtaaatgggctcctccctggtgaccacagcgtagagcctcacgagcttgtcatgctgcagggtcttcatgaggttggcttcttccaggaaggcttgcacagacatagttcctggcttcagggttttcacagccaccttggtactgttgttatagtaacccatccagacttccccaaactgcccagcgccaagccttttcaccaacttgatggactcccgggggatctcccaggcatctttatcccatggcttctgtggcttgggactaatacaagccttctccaatcttctgcacaagccatctgcctgcttttggtaatgtttaatcatgtcgctgatacagggaaaagtgattcgtggagagatgtaatagcccccattatccagacttctaattttgtagtgcttaataacatcaccatgcacagggtcaaagtctctgacagacagagagaagcttccttttaatgtttcactttctctaataaggaaagctccagcgctatttcctggtgccaaaagctgcctttctgcgtccttcctggttatatccttgaaaaaccactcttctgtttctaaggtgttgagtttggccacatagttgctggggatgaagccttctttttttgttaaaagggactttgctttccaccattctccatgctcctccaggactttcatcttctctcctttcttgaaagacaagtcgtccgggtggatgccatcataggggtacaaggctaccacaatgtctccttgttcctctggatctttagtttgaaacctctgtccaggtaaaagctgagattctggaactggcctttgctgtttattggacgttggatctctcacataaatagttctttcagtattacgtactggttgagtcttcaaatctactccatcgtcactcaagctgtctttcccttttgattttatacatcccatatttcccgctcgcggtgaaagtttcggggcggcggagctccacggtgacttgagttcagagtggggggcgcgacggggcggcccagcaggacctgcgtatggggaggctgctggccgggaacgctggacgcgcggcgaggggctgctggcgcggggccgggggtggcgcggccgccccgcttgccgcgggctggaggctgcagcgcgtctggcccggaggcgccacggccggggagcgagcggcagcgcggcccggcgcggcgggagaggaact

SEQ ID NO: 15827 - RNA, 4116 nt, Homo sapiens
  source 1..4116: mol_type = other RNA
gctgggattacaggcatgagccactgtgtctagctgactggagaagcttttaaaatagactgacatacatctcccgctgcacaacagctaagtcagaatcttggcggtagggagtatggattctgtctttccagttctctacaataacctgaggtgtgatgacatgagccattttgcacaccactggatacccgaaaatgctacaaacacctattcagcccctcattatgcctgtctgtcacagggaggctggaaacctatagctaagtaaggagactgtgtgtgctgttcatcaagggaacgtgtgacttccacacatgctggacaccagagatgaggcccaagctggtgaagggcccacatggaggtaaggatcacaggcttgattgggagggaaagacaagtggaaaatggcaagaagaggaggaactgggagaagcaaaacaaggcgaagataaatttaataattttctttaaataaatttgttatgctaaaaaaaaaacctctagtcattttctagagacttctttttgccttagggattctttatagttcctctccatgtaacatattgggtaatacttgtggttctgaaataaaatgcaagcaggggggtgtacacaaaaaccttaccactgaatcaagggaccagctgtgcagacattatgtaacagtaatattctatagttctgaacatggcacttgtgaatcaataattttagaatattttagaaaggacatttaaaaaaatcacataggaaacaaagttaaaatttagaaaaaagtagaatattttatcccatcttctaagcacctcaagcctaaacaaaacacacagaatgaaattttaatgatgcctgttaagcctatttgaaaacaaattctatctggcccccataaacggatgttcaggtgttcaggcaatcaactccttggttctccaatctgaaatgttcaaaggaaggaggtagaacttgggcaagtttaaagcatgtagctctgttgaatcacttctaaccaccccgcccccagctgatgaccaatttttacactgaccacagctgaaaatgtaaatgcaaataaaaagcttgagatgttattggacgaggtgtattaaaataaaatcaaaaatagaaatattaggtatatacacaacagcataagtgaaacacatcatgtgatacagaagtttccattcaaagcttacaggagaaaaatttagtgaacagaaccgcttgaacctcctgccaccgtggcttattagagccttgtagtcacttatgttccttcatatccttgggtataaatagtctcatacacatgctacacaatttagaaaagattgctgaatcataaaaatagccccgaatgtggcactttagctttctagagtacaactaaaattaatacttgatctttaacataatgttcaaatatttgaagcaacaaaggaaactcttatgttttagaaggccctataaggttcttcagagattagaatcttagttcttccaaactacattgtcaaaacaaatctggatataggaaattgtggaaatgaaaaagctggactcttaaaaatattccttctaaacacagagcagtttctgaggctcttctccctttcctgggaggtccaggtgagcccggtgccttcgggtgagcagacagggcagctgtgcgtgctcacgggctcctcctgctggaagagagagagatgtgcacgccactcctatggcatgtctagcaggtctgagcagtgttcatagaagaaaaatgttttaacagtctcagattttgggaggtagggggaaaaaaatcattgaaatctgggaaagacatttttaagctgctgacttcacctgcaaaatctaacaggttggattagtttttttttttttttaaacaagtaagccaaagcacaaagaaatgtcatgctatgtatatatccggttattttagctttataaatgagtttagttctgcaattattggggattcattgcaatggtctctgaaactttgagtcctatgtccatttgtaaacatagagctagttgggtgcatttttggagagaatagatgttttcttctcaaacggctgcactcagatgttgtcaagcagagcaagattaccagctgctgaggacaagtccaagttgcaactgagtggagaatccatctaagagtacagaatactttcccatttagagggtgttcttcctgagtaatttagcctctatttcaggatccaggcacggcagatgatccccgcacatgaaatcataagtgcaaccagtgatggttacttttcctctctaaatgaggcagccacccctgccaaatggacgggtctccctgtgctctaaggctgctgctggtattgcccttccgtggctgtgtagaaatcatccaggacgctctgtaagtagtcaaacgttggtctctcttctgccttttctttccagcacattttcataatgtcatagagctcatctgggcagttctccacacggggcatcctgtagccctgggacagggcggtcatcacgtcggcattagttctccctgggtagggaattttcccataggtgacaatttcgtataggaggattccaaaggaccacacatcagacttaatagtgaaacatccaaagttgattgcttctggagccgtccacttaatagggaacttagcaccttcccttgctgtgtactcattatcttcaattactctagcaaggccaaaatctgcaattttgcacatgagtgactcggagaccagaacattagctgctcgcaggtcccggtgaatgtagttcttccgctcgatgtatgccattccctctgcaatctgagcagaaaagtcaatgagctttggaagcagcactttgccaccttcatcgctcttcaggaaatccagcaaactgcccttggccatgtactcggtgatgatgtaaatgggctcctccctggtgaccacagcgtagagcctcacgagcttgtcatgctgcagggtcttcatgaggttggcttcttccaggaaggcttgcacagacatagttcctggcttcagggttttcacagccaccttggtactgttgttatagtaacccatccagacttccccaaactgcccagcgccaagccttttcaccaacttgatggactcccgggggatctcccaggcatctttatcccatggcttctgtggcttgggactaatacaagccttctccaatcttctgcacaagccatctgcctgcttttggtaatgtttaatcatgtcgctgatacagggaaaagtgattcgtggagagatgtaatagcccccattatccagacttctaattttgtagtgcttaataacatcaccatgcacagggtcaaagtctctgacagacagagagaagcttccttttaatgtttcactttctctaataaggaaagctccagcgctatttcctggtgccaaaagctgcctttctgcgtccttcctggttatatccttgaaaaaccactcttctgtttctaaggtgttgagtttggccacatagttgctggggatgaagccttctttttttgttaaaagggactttgctttccaccattctccatgctcctccaggactttcatcttctctcctttcttgaaagacaagtcgtccgggtggatgccatcataggggtacaaggctaccacaatgtctccttgttcctctggatctttagtttgaaacctctgtccaggtaaaagctgagattctggaactggttgagtcttcaaatctactccatcgtcactcaagctgtctttcccttttgattttatacatcccatatttcccgctcgcggtgaaagtttcggggcggcggagctccacggtgacttgagttcagagtggggggcgcgacggggcggcccagcaggacctgcgtatggggaggctgctggccgggaacgctggacgcgcggcgaggggctgctggcgcggggccgggggtggcgcggccgccccgcttgccgcgggctggaggctgcagcgcgtctggcccggaggcgccacggccggggagcgagcggcagcgcggcccggcgcggcgggagaggaact

SEQ ID NO: 15828 - RNA, 3667 nt, Homo sapiens
  source 1..3667: mol_type = other RNA
gctgggattacaggcatgagccactgtgtctggccacataaattttcagttcaattcaacaaacatctactgggtttcattagagggaccatcaatccttttattgacaccattaactcccaacaatcttataggtaaatctgggttttcttatcttaggtttacttatagtaaggtacttggtaagaagataaaatgtttcctattcttcatttatattgtaagtcatctgcatgcttatctagaatttcaacttacaatttgcctggtacattgttaccctactctgattcttagaggagcccaataaccatatccattcttcgtgtaagaaactgtcactgttgaaaagggactccaaatgtgcataaaagataatctcaaaaccaatggttgcaaaatgaaacatgaacagtcaagctgcctctttaacacaggcatttacaattaggttgccttcagtttggaaacctctgtttagtttccctgcaacacagatttaatgtccatccctatctagtgctttaaaacacacacatacaggccaggcatggtggctcatgctgtaatcccagcactctggaaggccaaggcaggcggatcacctgaggtcaggagttcaagaccagacaggccaatgtggcaaaaccctgtctctactaaaaatacaaaaaaatgagctgggtgtggtgtacctgtagtcccagctagttgggaggctgaggcagaagaatcacttgaacccaggaggcagaggttacagtgagcagaggtcacgccactgcactccagcctgggtgacagagtgagactctctcaagaacaaaaacaaaaacaaaaccacacacatatataaggtcaaaaatcctttacatttctgttttctcaaagtaatatcttcccccaaccccttggacatttctgctatggtattattggaaaacctcaaaattgtattttagggtttctggagtccatggagaatccctaacccatatcataaaacataaaatatataataaaacataacccatatcataaaacataaaattctctctggattaatgttgttgaactatatgtgaaaggtgggaattataaactgaaccctctagagtttaccctgaaaggctaaacacacagatgacctggagtggaggcaggaaccaacgtaccacattttttgtacaaattgttggcagttcttaaagggacagaagattactgtttacattttgcagtctcttgcttttttaagacaatttcatgaatgataaaagtgatgtcgggaagacataaacctgaaactccaacccccatcctcgctcttttattttgttttaaatcatcatatagtaatttgagtttaagactaacttcagccattcagaataatattgaaagtatttcctaaatcatttaataacagtgaccacaataaataaagatttggttctaagattacaaataatgaaaaatgttaactttgagattcaaaaccctgtagcatctggaaaaggttgtttataaagtataatcataacaataacattaagacttatgtgtgaaataaaacatttctgaaacacttaggaatacatgcttattccacttttgggataactactagtacttcctgaaatctgttgggtagtaatttctgtaaaaagaaagcagcaattccagaagctgggtgtcgagattattatacataataaaaaaaattcagttttccagcactggcttaatataaaatggccttaaaaagtatttttaaatgcaaatattgaattcttgatgcttcctttaagacacgtactctgtcaagttaatgaagtatgatcttggattgtcttctatgaggtatctgtagagtcacatctcattctgtaaacagtgtttgggaaacatcttcatctgaaaattatggcaaagtctccttttaccattaaacagagactagcactgtcaggctggggcaactgtttgagagactgatgcttgatacggacacagctgtcagggattccattttctcatttaggtttgcatttattgctctcaagtctgtgactgcaggataaataaggcaggagttcccaaaatacataaaattagggactagaactctgacaatttgcacaagttctgtccacttcttgcctgtaactctgaagctgaatagtacatctatacatgccaaatgtgttcaataataaatggtttgctttggactgtacttcctcccatttagatgaacttccaggaattagctgtatgtgaactatggcagtagattttcctgaagtgagagaccagatatttaaatcttcgactgaatatacatcttctattttcatcaaggcttctttgatatagtctacattcaaatggcttggcacaccttctagtattataactactgtatcccatatgattcgaaatgttgtaaaagccacaagtaatgaaaatacgtatgtacagatggggtcagcaatcttgtattctggcttgaatcgtatgatgtatgcagctattagcacaccaacactctgtaccaaatctcccaaagcatgtacaaatgcagctctcactgccaggctatcctgcccatggttacgttcacacccagaacctctggtaggggaatttgaaggcagggagtgggaatgggagtgacggtgaccagactggttcaacagaaaccccattattacattaactgcaactccaacagctgcggtgatgagcattatatctccatttatttcatagttcatatggatagttctttgcacagcttcatataagaggaatcccataagtatatacaccaacagcacactaatcatagctgacaaaacctctaagcgatgaaatccaaaggtgaatcttttggttggtgattttgatgatagccacaaagcaagcagggtgagtatgatggcgcttaggtcagttaacatatgaagtgcatctgtcatgattgctaggctatttgcaatgtatccacctacaagttctccaatcatgaaaagcaagtacagaacggcagcaatggtcaacctggctttcacctttctctgcttcagtatctctctctgtttgctgcagttgtcacaggagtccaccttcaaactcagctgactgttggtcaaaggtaagtcttggtccagtaaggaatcatcgtcggcctggagggtcgggtgcgccccgttaacaggcctttccggggcttcggaaccgtcatcggccaccacaactcgaagtttgttgaaccgagaaagcccctcgtcccccgcctcatccgagaagtcaaaggcgctggtgtcatttaaaaacagcggcgcatcatccttccttagcatagatttgaggcgcttccacgcgccagagccggccatggcagaggctgagcggccgcggtgcggaacggcttgggggaggcggacggccggcggcgcctacttcaccggagcgccagttctcgagggcagtgccgcgcgtccctccccatcctggggcgctgccgcggggccgcaactcatctccccgcccccggccggctcagcgaggcgggctcgcgctgctccacccgcggccgcaggagagtggggtcgtgctcgcgcccgccgcgcccgctgctggaggccggctccccaggtct

SEQ ID NO: 15829 - RNA, 3522 nt, Homo sapiens
  source 1..3522: mol_type = other RNA
gctgggattacaggcatgagccactgtgtctggccacataaattttcagttcaattcaacaaacatctactgggtttcattagagggaccatcaatccttttattgacaccattaactcccaacaatcttataggtaaatctgggttttcttatcttaggtttacttatagtaaggtacttggtaagaagataaaatgtttcctattcttcatttatattgtaagtcatctgcatgcttatctagaatttcaacttacaatttgcctggtacattgttaccctactctgattcttagaggagcccaataaccatatccattcttcgtgtaagaaactgtcactgttgaaaagggactccaaatgtgcataaaagataatctcaaaaccaatggttgcaaaatgaaacatgaacagtcaagctgcctctttaacacaggcatttacaattaggttgccttcagtttggaaacctctgtttagtttccctgcaacacagatttaatgtccatccctatctagtgctttaaaacacacacatacaggccaggcatggtggctcatgctgtaatcccagcactctggaaggccaaggcaggcggatcacctgaggtcaggagttcaagaccagacaggccaatgtggcaaaaccctgtctctactaaaaatacaaaaaaatgagctgggtgtggtgtacctgtagtcccagctagttgggaggctgaggcagaagaatcacttgaacccaggaggcagaggttacagtgagcagaggtcacgccactgcactccagcctgggtgacagagtgagactctctcaagaacaaaaacaaaaacaaaaccacacacatatataaggtcaaaaatcctttacatttctgttttctcaaagtaatatcttcccccaaccccttggacatttctgctatggtattattggaaaacctcaaaattgtattttagggtttctggagtccatggagaatccctaacccatatcataaaacataaaatatataataaaacataacccatatcataaaacataaaattctctctggattaatgttgttgaactatatgtgaaaggtgggaattataaactgaaccctctagagtttaccctgaaaggctaaacacacagatgacctggagtggaggcaggaaccaacgtaccacattttttgtacaaattgttggcagttcttaaagggacagaagattactgtttacattttgcagtctcttgcttttttaagacaatttcatgaatgataaaagtgatgtcgggaagacataaacctgaaactccaacccccatcctcgctcttttattttgttttaaatcatcatatagtaatttgagtttaagactaacttcagccattcagaataatattgaaagtatttcctaaatcatttaataacagtgaccacaataaataaagatttggttctaagattacaaataatgaaaaatgttaactttgagattcaaaaccctgtagcatctggaaaaggttgtttataaagtataatcataacaataacattaagacttatgtgtgaaataaaacatttctgaaacacttaggaatacatgcttattccacttttgggataactactagtacttcctgaaatctgttgggtagtaatttctgtaaaaagaaagcagcaattccagaagctgggtgtcgagattattatacataataaaaaaaattcagttttccagcactggcttaatataaaatggccttaaaaagtatttttaaatgcaaatattgaattcttgatgcttcctttaagacacgtactctgtcaagttaatgaagtatgatcttggattgtcttctatgaggtatctgtagagtcacatctcattctgtaaacagtgtttgggaaacatcttcatctgaaaattatggcaaagtctccttttaccattaaacagagactagcactgtcaggctggggcaactgtttgagagactgatgcttgatacggacacagctgtcagggattccattttctcatttaggtttgcatttattgctctcaagtctgtgactgcaggataaataaggcaggagttcccaaaatacataaaattagggactagaactctgacaatttgcacaagttctgtccacttcttgcctgtaactctgaagctgaatagtacatctatacatgccaaatgtgttcaataataaatggtttgctttggactgtacttcctcccatttagatgaacttccaggaattagctgtatgtgaactatggcagtagattttcctgaagtgagagaccagatatttaaatcttcgactgaatatacatcttctattttcatcaaggcttctttgatatagtctacattcaaatggcttggcacaccttctagtattataactactgtatcccatatgattcgaaatgttgtaaaagccacaagtaatgaaaatacgtatgtacagatggggtcagcaatcttgtattctggcttgaatcgtatgatgtatgcagctattagcacaccaacactctgtaccaaatctcccaaagcatgtacaaatgcagctctcactgccaggctatcctgcccatggttacgttcacacccagaacctctggtaggggaatttgaaggcagggagtgggaatgggagtgacggtgaccagactggttcaacagaaaccccattattacattaactgcaactccaacagctgcggtgatgagcattatatctccatttatttcatagttcatatggatagttctttgcacagcttcatataagaggaatcccataagtatatacaccaacagcacactaatcatagctgacaaaacctctaagcgatgaaatccaaaggtgaatcttttggttggtgattttgatgatagccacaaagcaagcagggtgagtatgatggcgcttaggtcagttaacatatgaagtgcatctgtcatgattgctaggctatttgcaatgtatccacctacaagttctccaatcatgaaaagcaagtacagaacggcagcaatggtcaacctggctttcacctttctctgcttcagtatctctctctgtttgctgcagttgtcacaggagtccaccttcaaactcagctgactgttggtcaaaggtaagtcttggtccagtaaggaatcatcgtcggcctggagggtcgggtgcgccccgttaacaggcctttccggggcttcggaaccgtcatcggccaccacaactcgaagtttgttgaaccgagaaagcccctcgtcccccgcctcatccgagaagtcaaaggcgctggtgtcatttaaaaacagcggcgcatcatccttccttagcatagatttgaggcgcttccacgcgccagagccggccatggcagaggctgagcggccgcggtgcggaacggcttgggggaggcggacggccggcggcgcctacttcaccggagcgccagttctcgagggcagtgccgcgcgtccctccccatcctgt

SEQ ID NO: 15830 - RNA, 4290 nt, Homo sapiens
  source 1..4290: mol_type = other RNA
gctgggattacaggcatgagccactgtgtctggccacataaattttcagttcaattcaacaaacatctactgggtttcattagagggaccatcaatccttttattgacaccattaactcccaacaatcttataggtaaatctgggttttcttatcttaggtttacttatagtaaggtacttggtaagaagataaaatgtttcctattcttcatttatattgtaagtcatctgcatgcttatctagaatttcaacttacaatttgcctggtacattgttaccctactctgattcttagaggagcccaataaccatatccattcttcgtgtaagaaactgtcactgttgaaaagggactccaaatgtgcataaaagataatctcaaaaccaatggttgcaaaatgaaacatgaacagtcaagctgcctctttaacacaggcatttacaattaggttgccttcagtttggaaacctctgtttagtttccctgcaacacagatttaatgtccatccctatctagtgctttaaaacacacacatacaggccaggcatggtggctcatgctgtaatcccagcactctggaaggccaaggcaggcggatcacctgaggtcaggagttcaagaccagacaggccaatgtggcaaaaccctgtctctactaaaaatacaaaaaaatgagctgggtgtggtgtacctgtagtcccagctagttgggaggctgaggcagaagaatcacttgaacccaggaggcagaggttacagtgagcagaggtcacgccactgcactccagcctgggtgacagagtgagactctctcaagaacaaaaacaaaaacaaaaccacacacatatataaggtcaaaaatcctttacatttctgttttctcaaagtaatatcttcccccaaccccttggacatttctgctatggtattattggaaaacctcaaaattgtattttagggtttctggagtccatggagaatccctaacccatatcataaaacataaaatatataataaaacataacccatatcataaaacataaaattctctctggattaatgttgttgaactatatgtgaaaggtgggaattataaactgaaccctctagagtttaccctgaaaggctaaacacacagatgacctggagtggaggcaggaaccaacgtaccacattttttgtacaaattgttggcagttcttaaagggacagaagattactgtttacattttgcagtctcttgcttttttaagacaatttcatgaatgataaaagtgatgtcgggaagacataaacctgaaactccaacccccatcctcgctcttttattttgttttaaatcatcatatagtaatttgagtttaagactaacttcagccattcagaataatattgaaagtatttcctaaatcatttaataacagtgaccacaataaataaagatttggttctaagattacaaataatgaaaaatgttaactttgagattcaaaaccctgtagcatctggaaaaggttgtttataaagtataatcataacaataacattaagacttatgtgtgaaataaaacatttctgaaacacttaggaatacatgcttattccacttttgggataactactagtacttcctgaaatctgttgggtagtaatttctgtaaaaagaaagcagcaattccagaagctgggtgtcgagattattatacataataaaaaaaattcagttttccagcactggcttaatataaaatggccttaaaaagtatttttaaatgcaaatattgaattcttgatgcttcctttaagacacgtactctgtcaagttaatgaagtatgatcttggattgtcttctatgaggtatctgtagagtcacatctcattctgtaaacagtgtttgggaaacatcttcatctgaaaattatggcaaagtctccttttaccattaaacagagactagcactgtcaggctggggcaactgtttgagagactgatgcttgatacggacacagctgtcagggattccattttctcatttaggtttgcatttattgctctcaagtctgtgactgcaggataaataaggcaggagttcccaaaatacataaaattagggactagaactctgacaatttgcacaagttctgtccacttcttgcctgtaactctgaagctgaatagtacatctatacatgccaaatgtgttcaataataaatggtttgctttggactgtacttcctcccatttagatgaacttccaggaattagctgtatgtgaactatggcagtagattttcctgaagtgagagaccagatatttaaatcttcgactgaatatacatcttctattttcatcaaggcttctttgatatagtctacattcaaatggcttggcacaccttctagtattataactactgtatcccatatgattcgaaatgttgtaaaagccacaagtaatgaaaatacgtatgtacagatggggtcagcaatcttgtattctggcttgaatcgtatgatgtatgcagctattagcacaccaacactctgtaccaaatctcccaaagcatgtacaaatgcagctctcactgccaggctatcctgcccatggttacgttcacacccagaacctctggtaggggaatttgaaggcagggagtgggaatgggagtgacggtgaccagactggttcaacagaaaccccattattacattaactgcaactccaacagctgcggtgatgagcattatatctccatttatttcatagttcatatggatagttctttgcacagcttcatataagaggaatcccataagtatatacaccaacagcacactaatcatagctgacaaaacctctaagcgatgaaatccaaaggtgaatcttttggttggtgattttgatgatagccacaaagcaagcagggtgagtatgatggcgcttaggtcagttaacatatgaagtgcatctgtcatgattgctaggctatttgcaatgtatccacctacaagttctccaatcatgaaaagcaagtacagaacggcagcaatggtcaacctggctttcacctttctctgcttcagtatctctctctgtttgctgcagttgtcacaggagtccaccttcaaactcagctgactgttggtcaaaggtaagtcttggtccagtaaggaatcatcgtcggcctggagggtcgggtgcgccccgttaacaggcctttccggggcttcggaaccgtcatcggccaccacaactcgaagtttgttgaaccgagaaagcccctcgtcccccgcctcatccgagaagtcaaaggcgctggtgtcatttaaaaacagcggcgcatcatccttccttagcatagatttgaggcgcttccacgcgccagagccggccatggcagaggctgagcggccgcggtgcggaacggcttgggggaggcggacggccggcggcgcctacttcaccggagcgccagttctcgagggcagtgccgcgcgtccctccccatctggccaactgaggggactttgggcggcctcttccaccttcccaggctgggaggcaagtgcggtcggagggtcacgccgggggctgggcgttgctgctaggagttccctccaccgaaagtgtgtctcaggaatctcgggtcgggatctgggttgcgggtgctcggcagaagacaaacccagcacttttcttgctaactgaaaaggcaagcagcttttctctcctcgaattgcttgtctctggcaaattggcaacatttgctgcagtcaactggagagggcaaggctgtcgtcgtcagcagttctgtgtcctactgtttttcagcaaatatgtattgtcctctttgtgctctctgccgtgttccttttgcctccaaggtatttacgatatggactaaactcaagcatagaaaatctagtacaggcataccttggagatactgcgaatttggttccagaccaccgcaatatgacaaagtgaggtctcacaaatgtttcatgtcccagtgcaaatacaatcatgtttataatgtagtctattaagcgtgtaatagcgttatgtctaaaacaatgtgcataccttaatttaaaatattgggagagaggaaggaaaaagtatatatacatttgttaattgctctgaggaaggagggtcgcatgagcccagaggttcgagattacagtgagctatgattgtgcctccgcacccctgcctggcgacagagtgagaccttgtctctaaaaataaacaagtaaataaaatacatgactgcta

SEQ ID NO: 15831 - RNA, 5417 nt, Homo sapiens
  source 1..5417: mol_type = other RNA
gctgggattacaggcatgagccactgtgtctggtcatctgttccctttctaaattgttcactgtgcagttatatgaagagtactttcctctgtcagttcacttttgggcataatatccttaagttgtggcctatttatcacaaatatttcaacatggttcttagacacttcaacagaccttctatcaaacaaaggttacagataacttttaaattagatggaaataaaaccgcaggcattcaagttgttatagttttaaaagagcaattatttatatttttcctacttaattcagctatacctggaaagaacgtatcttgggcaaaaatgtcaagttagaacatttgcattctgatcaactatgaaatttatcctagttacatactaaagtgactcagaaaaagtaagtgaggatttgcttaaaaaatgattagccagaatagaccatatttggggacacaattcgttttaaaattaggtatgaaatgaagatttgtttattcttggcaagattcctttttaatttgcaaagattgaaaagagaaattttggtttttgcttctcaaattagcagagtcatgattgttttcttcagatttgcaatgtacattttagctagttttaatgaagacaaattcttctcaatcaggagtttcccattcattaagtgagacagatgacagccttggtatattttgttagagccagcctcttgaaactggctgcctcccttatttaggtctataggaataacagggcttatttttctgaaggaaaaatcaaagaagtcaatattttgctagggcaaagtgtcgagtatcttcaaaacaaatgagccaaccacctcccagatttgaagtggtaagaaagtgtgttttcatttttctcatttgagggacacataccctcactttatgtggtaggtggaaggctaagatacttggggatatacacatttagagattttcctaagagatgtttgagatttctctgatgtgtgctattccacaacccaagacattttgtgtcctttggtaattctctaaccctccctgtaactcccttgcttagattttgatggctttgaaacatgaccagaagctcaaataaagaaaaagtaagctcgaaagcatcccagcttcctgcggtgctgcacgaggtcagcagaagacgcttaagaaaggatgcatcattcacacaagatagaaggcacggcctgaggaagggctggccaaggtttacaagactcagtgctaaggtggctccaagaggaaaaacactggctttaaatgttcaccattccagtcagcactagaagctaaagagcagtggatgtcctatcttcagttttgccagggccacttctgaggagagctattgaatctagagctgcaccatctcttaagatagttaagattctgaccaatgaatgcaagctaagggatgcattcattttcccttactctgaccagacacacaattgcatatggagaagctgaggtttggcaagaacatacagtgcatgtagtgaccatgtctttgctgaaaaccctactggatacgcacaatgcagagtgcattctataagactggaggcaaaagcaataactgcaaatgctcatttccatggaacagtaactgtgacagtacttcattggaattacccagattaacgggtaattgccaagtattactgtacaactctgcacttctttttttccctttgtcttacagaagcatagccctcaaagagaaaccaggaagatgaaaggcagggagaagaaaagagagaagaggaggtggcagatcaatctaacttgtttctgatgagtggcaaatatccagaatgttaggacaatctttatggattgctgaggttggagattgaaacagttataacttcatatttaagtgaagaaagattaaaaatgaaaacatatacaccatattaaatagttgcctacattgaatattcatagacaaatcactaaggtaaggattttttcctcaaagctgttatctgcacttagactaagttcagactctgcagtgcctactagaactatgtacaaattcacgtgaagataaaatagaaacaaaatttagtatggttctattttgtgaaatgttaaccacattttatttgcatgtgtatgtgtgggggtaattaagtgacagtttaaaatatgtcaatactcattttatccttttttactgactctctacagttttgatgttttatcagctttttcaataatcgtaacaatactaacaataattattggcattagttttggaacttgaatattaatgttatttttaaattaaagcattttttagtttatttcaaatcatttaaacttgggcaaggttttcccagctgctttttaaaaaacagagtttgttgtttctgtgggctcttcatagcgcttgagtggaaagcaagagctccagacagggtacagaggagtgttttgacattattaataataatcacctcctttaattgtggagtgcttcactgtgtactgagaatttttttacatttttcgttaaattctcacctcacctttgggaggtagggatcatagttccacttcattgatgaggaaaactgtagtgcagagatggcaaacactgtccaagaacatggtggtggatgggacccaaaccccaacttttgctcccatgttctctgtccactggctatggctcttgcccctgtgtacagatacaggctctggacaagttcaccaaatcccttaggcttcagccccctcatctgcagaatagtggcttggattccaccatcttcaaggtccctgccagcttttctttatttgaatttggatttattaagcagaaaaaaaagtaatgggagtttgtgggtaccaatggattaaaggggtaaaatctggaggctagtgagtaaattaggtctccaaatggctcactgtggttgtgatgagcttggaggaatgaaggcaaactttgtcacattaaactctgattcttaacagagtctcatgaaacctataggctccgaaagaagaacaagaagaaaaaagactttcacacacatacaaatatttgtaacagttttaggtggttaatagacggacttcttagagatgcatgggctgagttaataaccacatattcacaactttctggcctatagggagcttcactgtggtcgttacacaaagtgagcaaaacttattttcatataaaaaatagtgattgagaagtgtgggcaaaagtgatgtgaaaagtgtatatattttatattgagaacagaccaaattatcagtgatgatgaaaattagcacagtggttgtctgtgagaatgtaggcattgcctgaaagagggcataagggaattttttaaagtgacggaaatgttctgcattttgattgaggccttggttacatgggtatgtacatttttcaaaactaatcaaatcgtaccattaatatttgtgcattttaccatatgtaagttttatgccagttaaaaaaatacaactgtgatgcgttttcaagacagtccttttttccacagataattgcttcccatatcattttcttggttattgggaaggggtaggagaaagaaaagctgatgttgctcacacgtgaatgtctcctttagaagtatttatagagaatgctacagcattttcaggcttcttttgaatatcctaagagaaaagttcctgactgcaggtctatgtttgtgatttctgtcccacaagcccatgagctgtatgtttaggtctgacagcagtgtcaggaatggaataatgagtagaaaatatggacctcagagacacccatattccctccaaaggggaaaggggttctactaatccttttactcttccatgtgcctacatatatatatatatcaggaaaaacaagatatgcacgaatctgaaaatttagattgccataatatcgttctgggttttaagaagtcaggaacaaaggaggactccatgttttgttttatgctgttgaaaaaatgacccatattcaatccaaaagctggatccattatttgtacctatttatcagctgtcacagggtctaccttggtggctgataaccacaggtaatgtctgctaaaacaaattcatcaggcctagaataacttcaacagtcagcagtgctgacttaacatctccacagcacacactgagatttctcttagaattgactgtagaaggttttcacagatttgctttttcattttgcatgcctcacattaaatattgttaaaaatttaaaaccaaattctgttttttcttttttttttttttttacaacttacaagtgttcatataagaagaaaacgactaaaaaaatacccacccaagcacctagaactcatctagagaacaatgctaataatacaaaggctgtgaccaaaatgctccatgattcgtgggaaagccaggaagcacagtctagcctctggaaggaatgtcaggcgggtcggatccaccgaggcgcgcagtcaatggtcctttgctccctaagtcaagttcagcagccgcatttctggttcaatgtcattacttatttcgactggtttaacaggctttaactcaacatgatcctggtagtaggagtgtgtatcaagtccacctatgaaatcaaatgtgtcttcttcttccatggaaatactgatcacataacaggcatacacaaaacccaccaaagagagtagtatttggacagcactgtggatgacctccaggtactggaagtcaacgatgcagcctgtgacagagacgtacgtgtaatcgtccatcatgccatgggctgagggaggcagcactcttctgacacaaccaggcccatgttctctccaccatgaccgatgtacagagatattgaatgtcattagatcggtgtcctttgagagtccacctacttccaaataaaagcagataatgaacacattccaggtgacccagagggcagtccacactgtatacaccattatgtatcgaggtctgtactgaatggtcccaaacaaacccaatatgacaactattatgtgtagaaaatttccaagaataggcgcccactggaaaccaaggaagtcaaagatctgcctctctaatgctgagaccaactgcagcgcgcagaggcagatgagcgagcagcgtccggtgcagcagcccatggtgccggcggcgtccgagcggcgctgactgccagagatcctcgtcctccgccgctgctgcctcctgactccggagtagtccccgcccggcccggcccaggctcctcggccccgcggccgccgctcgcggctccagggctcggggctcgcgcccgcctttgttagtttcccggcggggcgggccgaggtcagtgcggtgcgcacgacccgagcgtctggc

SEQ ID NO: 15832 - RNA, 4330 nt, Homo sapiens
  source 1..4330: mol_type = other RNA
gctgggattacaggcatgagccactgttcccagctggatttcttactctaagttacttatcttaaaaaaaaaatagtctaagattacaaattatcagttccagaagagatatacctaacacaaaaattaacctactaaattgaactatatgagtatcaatacaagcaacatgagtaagccttaaatttcatgtttttaaagcttacaaagggtgtaactaatttattcaactccaacactttattcttattacagaatcaaagcttttagacattaagaggaacaagggaggatctgaactattttaggtttaaaagcccatgatcagggatattaattgcagccataaataaactgctgaggccaaataaacaactgcattcctataatcgctgccaaaaacactgcatacatcctcaaacattgagacaaaggatggcagacaggtttcaactctaattgttaagtggctgcctccaacagaatattgagactggggaacaatgtggggcaggtttcaactctaattgttacgtggctgcctccaacagaatattgagactggggaacaaagtggggcaggtttcaactctaattgttacgtggctgcctccaacagaatattgagactggggaacaatgtggggcaggtttcaactctaattgttacgtggctgcctccaacagaatattgagactggggaacaacgtggggcaggtttcaactctaattgttatgtggctgcctccaacagtatattgagactggggaacaacgtggggcaggtttcaactctaattgttacgtggctgcctccaacagtatattgagactggggaacaacgtggggcaggtttcaactctaattgttacgtggctgcctccaacagaatattgagactggggaacaacgtggggcttgatgtcaaagagaactcagaaggattataaaagcctgtcgtgggcacaagaatgtggtaccttgtgctactcttggcttcagcattaagctgacaaagacttcctactgcaatacctgactttcgtttctattatgaacacgatatttcactgttgtttctcatcaaaagcacctgatgtcaatgtatcaaaatacagagatcatgaaattcttttttgctatgtccgacaaaatgaacaagaaactgaataccagttttctagatgcactaataaataacttcagttaaaataactagagttacattttttcaaatgctcttattcatctggaaaattcagtgttatatataaatgttacatatacatatgtgtgtatatatatatactgttttaggagaaaacagcatttcagtttgatattttaaatgccaattatgcacatttataatagtaagatttcccattaagtgaaacgttatagttacctataaacgttcatttttcactatttacaatttgaattatgtaatacttgcatactgcaactaattgttatagaagagtcacatagacaatataaatctgatgtccaatcctttacaaatacgaaatttgtttcactgggttttcaaactatcaagtataaataggaaaaggtcagcaatacttaggatgaggcactttaacaattactcagaaaggttaagtgtacaaaactgtaaaccaaaaccctgcatattaatcttatccttaatttcagatgtgattaatctgagatggtctatttaaggagtgttaagatcatcacagaccagttaatgtgcccatatacaaatgaactaaactatctaatgacacttgggtttcagaaagggactctttcaacactaaaacttctgtagaattttttcataaacaagtataaacacactgctctcacaaaggcaaatggtatctctaccatattcctagacaagaatgccctcaaatgtttaactgaatcacaattttacagtcttatgtactctttaaaaatagttttcaaaatactcagaaattttaaaattaaaactaccaatactttttagattacaattttaagataaaaaaggtaacgaataggtattttaccagccttttgtgaaagaccttttaaacatttctatttgagcacctcattttcaaccttaaatcatgttctctgtatatttacactgcacgttttggtagttcaggtaataaatacttgattaagggtaataattcccttttttttttggagacggagttttgctcttgtcgctcaggctggggcgcaatggcgcaatctcagctcactgcaacctctgcctcccgggttcagccgattcttctgtctcagcctcccaagtagctgggattacagacacccgccaccatgcctggctaatttttgtatttttagtagagacgaggtttcaccatgttggccaagctggactcgaactcctgacctctggtgattcgcccgccttggcctcccaaagtactgggattacagacattagccaccacacctggccaattcctgttttctgaattcactatgctgtattttttccccaactgtctgatttccacattcttctattagttaaaaaaaaaaaaaaaaaaaaaaaggctgactcaaattttaaagtttaccagaagagattaaaatcttgatatataccaagaaagaatctgtggacccattagctaagttttaggtaagagtagctaaatctcattaaacctgtttatttcttctaatttataatttgagtaatttccatagctcagatatacaaatgtcctttaataaaaatgcagtaataatttaacatggttagctgttccaggttcacttatcaaaataacttgccatgaatgtgtacacatgtacttcttaattccctagaacagtttctccttttctaaagaaactggctttcaatcaatatactaccagacacttaagtctctactaaaatcagaagttaaccagttttcaaatacatggaaagagaaaatactgatttagaaagacaaaaattaagcttggcaaaagtggtgacttttatttacaattgcatgtgtcaagattacaatggaaacactagtgataccatctgaacaaaagcaatgatttattggtaatggcaatgaatgaaacattgacagtctctggcgagaatcaagcaattatccaggagctgtagatctgattgcaatatggttgtccagtgtcttttgtaccttagtggctttctccttttttgccaactactcgtttgaagtcattcatatttgttgcctggactggagtaccaataaaagtaaaatatgaaattcttgttgtttcctcttcaccttgattcgactgaacaaatatagttacactgttaacattctgaaacttaacataacgaagtggaacaatgccatcttctttaatatcatcctctgtcagttccagagcttgagttggttcacttctttctgcctcttcaaaatccatagatcggggtaggttgataaaaatttttacatatttagggccctgaccattatctggcccttgaaatttcatggaataaagcttaacaggttgattgaatgccacagtaataagcagctgttcatcacagtcagattccaagaaggttgtgtcttttcgtaaacagttgtcaaatccatgctcatcactttcattaagacattcacaaccagctttgttaataaaaggcattaaatccatatagccttttggaatatctgtgtcctcattgcttccagggtcattttctaagtgctgcttgattttttcttctaatcccacagcatctgctccttgatattgatcaattctcactttgtttcgaaaaaacaaaaatgtaggtgttgctgatatattgttggtggcagctgttccctgaagcaattaataatgtgctactcttcttaactaatgcagccataatgacatctgtaataatgacatcaacataacatcttcctatcttcaaaggaataagtactgacactgatgtacatcgacttccaagaaaacagcctgtggatatttattactcatagaactgaatgctggggcaatcctcaaacatggcccacaccctctcatggtgaacttgaccacggcgagtctggagcccgcgccgctcagctctggctggaaatccgggtcgctcccgacgggcttcacccccaccatcctcacagagagcccggcagggtggccgcgacgccactggctttgaaactgaaggagaagacgatctgggagaggaaggagagatgctcaggaaggccgaggcctggacagaagaggtggcgaccgccgagtcttctcccgggactctcagt

SEQ ID NO: 15833 - RNA, 4225 nt, Homo sapiens
  source 1..4225: mol_type = other RNA
gctgggattacaggcatgagccactgttcccagctggatttcttactctaagttacttatcttaaaaaaaaaatagtctaagattacaaattatcagttccagaagagatatacctaacacaaaaattaacctactaaattgaactatatgagtatcaatacaagcaacatgagtaagccttaaatttcatgtttttaaagcttacaaagggtgtaactaatttattcaactccaacactttattcttattacagaatcaaagcttttagacattaagaggaacaagggaggatctgaactattttaggtttaaaagcccatgatcagggatattaattgcagccataaataaactgctgaggccaaataaacaactgcattcctataatcgctgccaaaaacactgcatacatcctcaaacattgagacaaaggatggcagacaggtttcaactctaattgttaagtggctgcctccaacagaatattgagactggggaacaatgtggggcaggtttcaactctaattgttacgtggctgcctccaacagaatattgagactggggaacaaagtggggcaggtttcaactctaattgttacgtggctgcctccaacagaatattgagactggggaacaatgtggggcaggtttcaactctaattgttacgtggctgcctccaacagaatattgagactggggaacaacgtggggcaggtttcaactctaattgttatgtggctgcctccaacagtatattgagactggggaacaacgtggggcaggtttcaactctaattgttacgtggctgcctccaacagtatattgagactggggaacaacgtggggcaggtttcaactctaattgttacgtggctgcctccaacagaatattgagactggggaacaacgtggggcttgatgtcaaagagaactcagaaggattataaaagcctgtcgtgggcacaagaatgtggtaccttgtgctactcttggcttcagcattaagctgacaaagacttcctactgcaatacctgactttcgtttctattatgaacacgatatttcactgttgtttctcatcaaaagcacctgatgtcaatgtatcaaaatacagagatcatgaaattcttttttgctatgtccgacaaaatgaacaagaaactgaataccagttttctagatgcactaataaataacttcagttaaaataactagagttacattttttcaaatgctcttattcatctggaaaattcagtgttatatataaatgttacatatacatatgtgtgtatatatatatactgttttaggagaaaacagcatttcagtttgatattttaaatgccaattatgcacatttataatagtaagatttcccattaagtgaaacgttatagttacctataaacgttcatttttcactatttacaatttgaattatgtaatacttgcatactgcaactaattgttatagaagagtcacatagacaatataaatctgatgtccaatcctttacaaatacgaaatttgtttcactgggttttcaaactatcaagtataaataggaaaaggtcagcaatacttaggatgaggcactttaacaattactcagaaaggttaagtgtacaaaactgtaaaccaaaaccctgcatattaatcttatccttaatttcagatgtgattaatctgagatggtctatttaaggagtgttaagatcatcacagaccagttaatgtgcccatatacaaatgaactaaactatctaatgacacttgggtttcagaaagggactctttcaacactaaaacttctgtagaattttttcataaacaagtataaacacactgctctcacaaaggcaaatggtatctctaccatattcctagacaagaatgccctcaaatgtttaactgaatcacaattttacagtcttatgtactctttaaaaatagttttcaaaatactcagaaattttaaaattaaaactaccaatactttttagattacaattttaagataaaaaaggtaacgaataggtattttaccagccttttgtgaaagaccttttaaacatttctatttgagcacctcattttcaaccttaaatcatgttctctgtatatttacactgcacgttttggtagttcaggtaataaatacttgattaagggtaataattcccttttttttttggagacggagttttgctcttgtcgctcaggctggggcgcaatggcgcaatctcagctcactgcaacctctgcctcccgggttcagccgattcttctgtctcagcctcccaagtagctgggattacagacacccgccaccatgcctggctaatttttgtatttttagtagagacgaggtttcaccatgttggccaagctggactcgaactcctgacctctggtgattcgcccgccttggcctcccaaagtactgggattacagacattagccaccacacctggccaattcctgttttctgaattcactatgctgtattttttccccaactgtctgatttccacattcttctattagttaaaaaaaaaaaaaaaaaaaaaaaggctgactcaaattttaaagtttaccagaagagattaaaatcttgatatataccaagaaagaatctgtggacccattagctaagttttaggtaagagtagctaaatctcattaaacctgtttatttcttctaatttataatttgagtaatttccatagctcagatatacaaatgtcctttaataaaaatgcagtaataatttaacatggttagctgttccaggttcacttatcaaaataacttgccatgaatgtgtacacatgtacttcttaattccctagaacagtttctccttttctaaagaaactggctttcaatcaatatactaccagacacttaagtctctactaaaatcagaagttaaccagttttcaaatacatggaaagagaaaatactgatttagaaagacaaaaattaagcttggcaaaagtggtgacttttatttacaattgcatgtgtcaagattacaatggaaacactagtgataccatctgaacaaaagcaatgatttattggtaatggcaatgaatgaaacattgacagtctctggcgagaatcaagcaattatccaggagctgtagatctgattgcaatatggttgtccagtgtcttttgtaccttagtggctttctccttttttgccaactactcgtttgaagtcattcatatttgttgcctggactggagtaccaataaaagtaaaatatgaaattcttgttgtttcctcttcaccttgattcgactgaacaaatatagttacactgttaacattctgaaacttaacataacgaagtggaacaatgccatcttctttaatatcatcctctgtcagttccagagcttgagttggttcacttctttctgcctcttcaaaatccatagatcggggtaggttgataaaaatttttacatatttagggccctgaccattatctggcccttgaaatttcatggaataaagcttaacaggttgattgaatgccacagtaataagcagctgttcatcacagtcagattccaagaaggttgtgtcttttcgtaaacagttgtcaaatccatgctcatcactttcattaagacattcacaaccagctttgttaataaaaggcattaaatccatatagccttttggaatatctgtgtcctcattgcttccagggtcattttctaagtgctgcttgattttttcttctaatcccacagcatctgctccttgatattgatcaattctcactttgtttcgaaaaaacaaaaatgtaggtgttgctgatatattgttggtggcagctgttccctgacactgatgtacatcgacttccaagaaaacagcctgtggatatttattactcatagaactgaatgctggggcaatcctcaaacatggcccacaccctctcatggtgaacttgaccacggcgagtctggagcccgcgccgctcagctctggctggaaatccgggtcgctcccgacgggcttcacccccaccatcctcacagagagcccggcagggtggccgcgacgccactggctttgaaactgaaggagaagacgatctgggagaggaaggagagatgctcaggaaggccgaggcctggacagaagaggtggcgaccgccgagtcttctcccgggactctcagt

SEQ ID NO: 15834 - RNA, 1682 nt, Homo sapiens
  source 1..1682: mol_type = other RNA
gctgggattacaggcatgagccactttgcctggcctctttttttcaatttttgtcaatattgaggaaattaaaacactttattatacccttcttaatcataccactagaagtgttttttctctgcctacctaaaaacccaaatccctaatacaccaattaccattaaagatagtttttaagaacgatgtcctagcagaggttatgcaagcaggctgctttaaaactgttgaaggccaggcacagtggctcatgccttgattatggtttgtgggctgtgtccccacccaaatctcatcttgaattgtactcgcataatccccacatgttgtgagagggacccggtgggagataactgaatcatgggagcggtttcccccatactttctcatggtagtgagtaagtatcacgagaactgatggttttataagggatatctgctttcatgtcttcctcatttcctgcttgccgctgccatctaagaagtgccttttgccttctaccataattgtgaggcatccccagccacatggaactgtgagtccaataaacctatttttcttcccagtcttaggtatgtctttatcagcagtgtgaaaatgaactaatacaagcctgtgatcccagcactttgggaagctgaggtgggaggatcccttgaggtcaggagttcgaaaccagcctggccaagaggatgaaaccccatctctacaaaaatacaaaaattagtcaggtgtggtagtgggcacctgtaatcccagccacttgggaggctgagacagaagaatcacttgaacctgggaggtggaagttgcagagagctgagcttgcatcactgcactccagtcagaggaagacttcatctcaaaaacaatacataaataaaattttaaaaaataaaactgttgggggcattagccacacgaacaactgtccaaaagccagggtctctggtttttgttgtttttgtttttacagttttattggttttatttaaaccccaataaaacaaacacattcactgtctattcactttctgcactgtgcaggctggcattggcattggtgactctgatgaccacctgggctgctctttccaagatggctttgcagttcttggaagaaacatcatgagtgatctcaacacagtaagatttgttgctcaccagcagtacttccagctccttaacgttgtggaccaggaacttccagaagccactgggcagtatgtgctttgtctttttgtttctcccataaccaatgttgggcatagatctggccctcaaaccttctatgaaccctgttgttaatacctctgtgtttccaccagttacccttaattttgacatatcagtctgactggttcccagtgaacttggtgctctttttgatgatcttgggcttcgcgagcggtctcaggatggccatgatggaggagatgggtgtcacctccataggcagtgccaaggaagacagctcaggtctttcttaatgaaaccgatatccttcgcgtactgacggaaacactggcggcacatattgaggccatatttccggatcagaccgtgccggtttgaacagacacgacaagagcgagaaccctggccgaattttcgcgggtggctccagtacagctgctggtgacccatcttgctctcagcagtgcaacgaggtaaaaggaag

SEQ ID NO: 15835 - RNA, 3552 nt, Homo sapiens
  source 1..3552: mol_type = other RNA
gctgggattacaggcatgagccagacctcatgagaactatcacaaggacagcaacaaggggatggtactaaaactttcttgagaaagccacccccatcatccaatcacctcccactaggctccacctccaatactggagattactacaattccacatgagacttcaaagggaaaggacaaatatacaagctatatgagtaagtataaattatttggggatcccagaggttaggacaacatctaacggcctttccacattgagtttagttgtaaggttctctccagcatgttttatctgatgtttagtgaggcctgagcgactaatgtaagatttgccacactcattacatttataaggtttttcactagaatgaattcgttggtgtttagtgaggcaagaccgccgcccaaacgccttgccacattccatacatttgtatggcttctctccagtatggtttctctgatggtaaaccaagtttgacctttcgataaaagctttaccacattcattacatttataaggtttctctccagtatgcatcatctgatgattaagcagaattgaacgtactctaaaggctttgccacactcattacatttgtaaggtttctctccagtatgaatactccaatgacgtgcgaggcctgagcgataacggaagaccttgccacattcattacatttgtaaggtttctctccagtatgaattctccgatgccttgccagggttgtagtggagttaaagactttcccacattcaatacatttgtatggcatctctccagtatgtcttctctgatggtacaccagacttgttttatgactaaaagttctaccacattcactacatttgtgtggtttctccccagtaggatttctgtgatatcttgcaagttttgaactttggataaaagcctcaccaaattcattacagtggtaagggttctctccagtatgaattaccagatgtttagtgaggcttgaacgctgagtataggctttgccacaatcattacatttataaggtttctctccggtatgaattttccgatgacgtgctaggcatgagtagtaactgaagaccttgccgcattcgttacactggaaaggtttctctccggtatgacttcgcctatgaattgaaaggtttccactgtcaatgaagaccttgccacacacattacatttgtaaggtttctctccggtatgcattctttgatgacgtgctaggcatgaatagtaagtgaagaccatgccacatttattacaatggagaggtttctctccagtatgacatctcatatgaaccgaaaggtatccaccgtaattaaagaccttgccacacacattacatttgtaaggtttctctccggtatgaattctctgatgtacagttagtaatgagccccaattaaaggctttgccacattcattacatttgtaaggtttctctccagtatgaactctctgatgcactgcaagatgtgaatgttgactgaagaccttgccacattcattacatttgtagggtttctctccagtatgaattctccggtgccctgcaagacgtgaacgttgaaagaagaccttgccacattcattacatttgtaaggtgtctctccagtatgaattatctggtgccttacaagttgtgaattctgataaaagaccttgccacatacatcacatgtatatggtttctttcctgcatggattatatgatgtgcagtgaggcttgagttccgtttaaaggttttgccacattcattacatttgtagggtttgtctccagtatgaactgtctgatgagttgcaagagaggaactttgactaaagcacttcccacatcgattacatttgtaaggtttctctccagtatgaattctctgatgaactgcaaggtgggaacttttactaaaggacttgccacattcattacatatgtagggtttgtctccagtgtgacttctccggtgatttacaagatctgaattttgtctgaagatcctgccacatacatcacattggtatggtttccctcttgtatggactatctgatgtactgttagtagtgagccccgatgaaaggctttaccagactcattgcatctgtaaggtttctctgtagtatgtatcatctgatgattaataagacttgaagacactctgaaggctttgccacactcattacctatgtaaggtttttccctaatatgtgttttctcgtcttgtgtaggtaacgaaagttgcaaaaaatcattcccatatttcctagaaatgttggtttggacaccaggaaaaattctttgaagtggtgaagctaaaaaacaattattaactgtcctctcaatttgattacatccataaattttctctgcagtttgaaatttctgcaattcacccagaccggactgaaaccttaatataagctgattttccatatgcttgttttctacgtccccttgactatgtcgaactctttgaccagtaagattgtttttatgggtcatcggcccttctttataatttatttcaccatctttccattgaaagtcaacttcctgtagatttttccggatttccctgaagtaaaaattttcagtgtcatagctttcatgtccttccaacatcactgcttggaatttttctcctgtgttactgttctgtattggtggtaattccttgatcacacatttaggagagataccggtgatcacgcctttcatgcattccccacagtttgggttcctcgctattttcacttggctcaccacagtccagggctctttcccttgctccaacatggagataatattcaggtcaggaagacagagtcccaggaagccgaggttcctgtagttctccaacatcacgtccctgtacaaagctttctgaacagggtccaggcatttccactcctcctgagagaattctacagccacatccctgaatgtcaaagatccctgaggaagagccatccctggctccttttctttcttctttctctcctgggcctctctctcagtcaatataattaattctttaaaagtcaaatcatagattgaggtgtgcgattcagttgcccgccatttcaagataaattaatctggtgtaaggaccacttgtaggcctagtgtggtggctcacatctgtaattccagtgcgttgagaggctgaggtggaaagactgcttgaggccaggaagtagaagctgcagtgagccgagatcatgccactgctctccagcctaggcggcagagagagaccatgtccccccccaaaacaaaacagaacaaagccaaaaaaaacaccaaagacatatcttgtagtgacagtcagtcatttcttgccccatttctcccctcctttatgctctactccatcattgggaagaagagagttaccacaaataactggatcaagtcactgccctctggctaaataggaattccaaatatcttttgatacaaatacatacaaaatgcacaaggcttatagaaaaaactttggtgattttcatcctcatgagtacaacttaaacatattt

SEQ ID NO: 15836 - RNA, 3443 nt, Homo sapiens
  source 1..3443: mol_type = other RNA
gctgggattacaggcatgagccagacctcatgagaactatcacaaggacagcaacaaggggatggtactaaaactttcttgagaaagccacccccatcatccaatcacctcccactaggctccacctccaatactggagattactacaattccacatgagacttcaaagggaaaggacaaatatacaagctatatgagtaagtataaattatttggggatcccagaggttaggacaacatctaacggcctttccacattgagtttagttgtaaggttctctccagcatgttttatctgatgtttagtgaggcctgagcgactaatgtaagatttgccacactcattacatttataaggtttttcactagaatgaattcgttggtgtttagtgaggcaagaccgccgcccaaacgccttgccacattccatacatttgtatggcttctctccagtatggtttctctgatggtaaaccaagtttgacctttcgataaaagctttaccacattcattacatttataaggtttctctccagtatgcatcatctgatgattaagcagaattgaacgtactctaaaggctttgccacactcattacatttgtaaggtttctctccagtatgaatactccaatgacgtgcgaggcctgagcgataacggaagaccttgccacattcattacatttgtaaggtttctctccagtatgaattctccgatgccttgccagggttgtagtggagttaaagactttcccacattcaatacatttgtatggcatctctccagtatgtcttctctgatggtacaccagacttgttttatgactaaaagttctaccacattcactacatttgtgtggtttctccccagtaggatttctgtgatatcttgcaagttttgaactttggataaaagcctcaccaaattcattacagtggtaagggttctctccagtatgaattaccagatgtttagtgaggcttgaacgctgagtataggctttgccacaatcattacatttataaggtttctctccggtatgaattttccgatgacgtgctaggcatgagtagtaactgaagaccttgccgcattcgttacactggaaaggtttctctccggtatgacttcgcctatgaattgaaaggtttccactgtcaatgaagaccttgccacacacattacatttgtaaggtttctctccggtatgcattctttgatgacgtgctaggcatgaatagtaagtgaagaccatgccacatttattacaatggagaggtttctctccagtatgacatctcatatgaaccgaaaggtatccaccgtaattaaagaccttgccacacacattacatttgtaaggtttctctccggtatgaattctctgatgtacagttagtaatgagccccaattaaaggctttgccacattcattacatttgtaaggtttctctccagtatgaactctctgatgcactgcaagatgtgaatgttgactgaagaccttgccacattcattacatttgtagggtttctctccagtatgaattctccggtgccctgcaagacgtgaacgttgaaagaagaccttgccacattcattacatttgtaaggtgtctctccagtatgaattatctggtgccttacaagttgtgaattctgataaaagaccttgccacatacatcacatgtatatggtttctttcctgcatggattatatgatgtgcagtgaggcttgagttccgtttaaaggttttgccacattcattacatttgtagggtttgtctccagtatgaactgtctgatgagttgcaagagaggaactttgactaaagcacttcccacatcgattacatttgtaaggtttctctccagtatgaattctctgatgaactgcaaggtgggaacttttactaaaggacttgccacattcattacatatgtagggtttgtctccagtgtgacttctccggtgatttacaagatctgaattttgtctgaagatcctgccacatacatcacattggtatggtttccctcttgtatggactatctgatgtactgttagtagtgagccccgatgaaaggctttaccagactcattgcatctgtaaggtttctctgtagtatgtatcatctgatgattaataagacttgaagacactctgaaggctttgccacactcattacctatgtaaggtttttccctaatatgtgttttctcgtcttgtgtaggtaacgaaagttgcaaaaaatcattcccatatttcctagaaatgttggtttggacaccaggaaaaattctttgaagtggtgaagctaaaaaacaattattaactgtcctctcaatttgattacatccataaattttctctgcagtttgaaatttctgcaattcacccagaccggactgaaaccttaatataagctgattttccatatgcttgttttctacgtccccttgactatgtcgaactctttgaccagtaagattgtttttatgggtcatcggcccttctttataatttatttcaccatctttccattgaaagtcaacttcctgtagatttttccggatttccctgaagtaaaaattttcagtgtcatagctttcatgtccttccaacatcactgcttggaatttttctcctgtgttactgttctgtattggtggtaattccttgatcacacatttaggagagataccggtgatcacgcctttcatgcattccccacagtttgggttcctcgctattttcacttggctcaccacagtccagggctctttcccttgctccaacatggagataatattcaggtcaggaagacagagtcccaggaagccgaggttcctgtagttctccaacatcacgtccctgtacaaagctttctgaacagggtccaggcatttccactcctcctgagagaattctacagccacatccctgaatgtcaaagatccctgaggaagagccatccctggctccttttctttcttctttctctcctgggcctctctctcagtcaatataattaattctttaaaagtcaaatcatagattgaggtgtgcgattcagttgcccgccatttcaagataaattaatctggtgtaaggaccacttgtaggcctagtgtggtggctcacatctgtaattccagtgcgttgagaggctgaggtggaaagactgcttgaggccaggaagtagaagctgcagtgagccgagatcatgccactgctctccagcttgggacgaaggggctgttgcgggtattttaaggtccgtagcgatccccaggtcacgggtatggagaaccgaggactgcgaagtgcacgtttaatcaaggtagacgaagagaagcaaacgtttaatccaggtagactgaaacacactcatagcgacgtggcctttccccagcgcgatctgcttccgggtgt

SEQ ID NO: 15837 - RNA, 3386 nt, Homo sapiens
  source 1..3386: mol_type = other RNA
gctgggattacaggcatgagccagacctcatgagaactatcacaaggacagcaacaaggggatggtactaaaactttcttgagaaagccacccccatcatccaatcacctcccactaggctccacctccaatactggagattactacaattccacatgagacttcaaagggaaaggacaaatatacaagctatatgagtaagtataaattatttggggatcccagaggttaggacaacatctaacggcctttccacattgagtttagttgtaaggttctctccagcatgttttatctgatgtttagtgaggcctgagcgactaatgtaagatttgccacactcattacatttataaggtttttcactagaatgaattcgttggtgtttagtgaggcaagaccgccgcccaaacgccttgccacattccatacatttgtatggcttctctccagtatggtttctctgatggtaaaccaagtttgacctttcgataaaagctttaccacattcattacatttataaggtttctctccagtatgcatcatctgatgattaagcagaattgaacgtactctaaaggctttgccacactcattacatttgtaaggtttctctccagtatgaatactccaatgacgtgcgaggcctgagcgataacggaagaccttgccacattcattacatttgtaaggtttctctccagtatgaattctccgatgccttgccagggttgtagtggagttaaagactttcccacattcaatacatttgtatggcatctctccagtatgtcttctctgatggtacaccagacttgttttatgactaaaagttctaccacattcactacatttgtgtggtttctccccagtaggatttctgtgatatcttgcaagttttgaactttggataaaagcctcaccaaattcattacagtggtaagggttctctccagtatgaattaccagatgtttagtgaggcttgaacgctgagtataggctttgccacaatcattacatttataaggtttctctccggtatgaattttccgatgacgtgctaggcatgagtagtaactgaagaccttgccgcattcgttacactggaaaggtttctctccggtatgacttcgcctatgaattgaaaggtttccactgtcaatgaagaccttgccacacacattacatttgtaaggtttctctccggtatgcattctttgatgacgtgctaggcatgaatagtaagtgaagaccatgccacatttattacaatggagaggtttctctccagtatgacatctcatatgaaccgaaaggtatccaccgtaattaaagaccttgccacacacattacatttgtaaggtttctctccggtatgaattctctgatgtacagttagtaatgagccccaattaaaggctttgccacattcattacatttgtaaggtttctctccagtatgaactctctgatgcactgcaagatgtgaatgttgactgaagaccttgccacattcattacatttgtagggtttctctccagtatgaattctccggtgccctgcaagacgtgaacgttgaaagaagaccttgccacattcattacatttgtaaggtgtctctccagtatgaattatctggtgccttacaagttgtgaattctgataaaagaccttgccacatacatcacatgtatatggtttctttcctgcatggattatatgatgtgcagtgaggcttgagttccgtttaaaggttttgccacattcattacatttgtagggtttgtctccagtatgaactgtctgatgagttgcaagagaggaactttgactaaagcacttcccacatcgattacatttgtaaggtttctctccagtatgaattctctgatgaactgcaaggtgggaacttttactaaaggacttgccacattcattacatatgtagggtttgtctccagtgtgacttctccggtgatttacaagatctgaattttgtctgaagatcctgccacatacatcacattggtatggtttccctcttgtatggactatctgatgtactgttagtagtgagccccgatgaaaggctttaccagactcattgcatctgtaaggtttctctgtagtatgtatcatctgatgattaataagacttgaagacactctgaaggctttgccacactcattacctatgtaaggtttttccctaatatgtgttttctcgtcttgtgtaggtaacgaaagttgcaaaaaatcattcccatatttcctagaaatgttggtttggacaccaggaaaaattctttgaagtggtgaagctaaaaaacaattattaactgtcctctcaatttgattacatccataaattttctctgcagtttgaaatttctgcaattcacccagaccggactgaaaccttaatataagctgattttccatatgcttgttttctacgtccccttgactatgtcgaactctttgaccagtaagattgtttttatgggtcatcggcccttctttataatttatttcaccatctttccattgaaagtcaacttcctgtagatttttccggatttccctgaagtaaaaattttcagtgtcatagctttcatgtccttccaacatcactgcttggaatttttctcctgtgttactgttctgtattggtggtaattccttgatcacacatttaggagagataccggtgatcacgcctttcatgcattccccacagtttgggttcctcgctattttcacttggctcaccacagtccagggctctttcccttgctccaacatggagataatattcaggtcaggaagacagagtcccaggaagccgaggttcctgtagttctccaacatcacgtccctgtacaaagctttctgaacagggtccaggcatttccactcctcctgagagaattctacagccacatccctgaatgtcaaagatccctgaggaagagccatccctggctccttttctttcttctttctctcctgggcctctctctcagtcaatataattaattctttaaaagtcaaatcatagattgaggtgtgcgattcagttgcccgccatttcaagataaattaatctggtgtaaggaccacttgtaggcctagtgtggtggctcacatctgtaattccagtgcgttgagaggctgaggtggaaagactgttgggacgaaggggctgttgcgggtattttaaggtccgtagcgatccccaggtcacgggtatggagaaccgaggactgcgaagtgcacgtttaatcaaggtagacgaagagaagcaaacgtttaatccaggtagactgaaacacactcatagcgacgtggcctttccccagcgcgatctgcttccgggtgt

SEQ ID NO: 15838 - RNA, 3317 nt, Homo sapiens
  source 1..3317: mol_type = other RNA
gctgggattacaggcatgagccagacctcatgagaactatcacaaggacagcaacaaggggatggtactaaaactttcttgagaaagccacccccatcatccaatcacctcccactaggctccacctccaatactggagattactacaattccacatgagacttcaaagggaaaggacaaatatacaagctatatgagtaagtataaattatttggggatcccagaggttaggacaacatctaacggcctttccacattgagtttagttgtaaggttctctccagcatgttttatctgatgtttagtgaggcctgagcgactaatgtaagatttgccacactcattacatttataaggtttttcactagaatgaattcgttggtgtttagtgaggcaagaccgccgcccaaacgccttgccacattccatacatttgtatggcttctctccagtatggtttctctgatggtaaaccaagtttgacctttcgataaaagctttaccacattcattacatttataaggtttctctccagtatgcatcatctgatgattaagcagaattgaacgtactctaaaggctttgccacactcattacatttgtaaggtttctctccagtatgaatactccaatgacgtgcgaggcctgagcgataacggaagaccttgccacattcattacatttgtaaggtttctctccagtatgaattctccgatgccttgccagggttgtagtggagttaaagactttcccacattcaatacatttgtatggcatctctccagtatgtcttctctgatggtacaccagacttgttttatgactaaaagttctaccacattcactacatttgtgtggtttctccccagtaggatttctgtgatatcttgcaagttttgaactttggataaaagcctcaccaaattcattacagtggtaagggttctctccagtatgaattaccagatgtttagtgaggcttgaacgctgagtataggctttgccacaatcattacatttataaggtttctctccggtatgaattttccgatgacgtgctaggcatgagtagtaactgaagaccttgccgcattcgttacactggaaaggtttctctccggtatgacttcgcctatgaattgaaaggtttccactgtcaatgaagaccttgccacacacattacatttgtaaggtttctctccggtatgcattctttgatgacgtgctaggcatgaatagtaagtgaagaccatgccacatttattacaatggagaggtttctctccagtatgacatctcatatgaaccgaaaggtatccaccgtaattaaagaccttgccacacacattacatttgtaaggtttctctccggtatgaattctctgatgtacagttagtaatgagccccaattaaaggctttgccacattcattacatttgtaaggtttctctccagtatgaactctctgatgcactgcaagatgtgaatgttgactgaagaccttgccacattcattacatttgtagggtttctctccagtatgaattctccggtgccctgcaagacgtgaacgttgaaagaagaccttgccacattcattacatttgtaaggtgtctctccagtatgaattatctggtgccttacaagttgtgaattctgataaaagaccttgccacatacatcacatgtatatggtttctttcctgcatggattatatgatgtgcagtgaggcttgagttccgtttaaaggttttgccacattcattacatttgtagggtttgtctccagtatgaactgtctgatgagttgcaagagaggaactttgactaaagcacttcccacatcgattacatttgtaaggtttctctccagtatgaattctctgatgaactgcaaggtgggaacttttactaaaggacttgccacattcattacatatgtagggtttgtctccagtgtgacttctccggtgatttacaagatctgaattttgtctgaagatcctgccacatacatcacattggtatggtttccctcttgtatggactatctgatgtactgttagtagtgagccccgatgaaaggctttaccagactcattgcatctgtaaggtttctctgtagtatgtatcatctgatgattaataagacttgaagacactctgaaggctttgccacactcattacctatgtaaggtttttccctaatatgtgttttctcgtcttgtgtaggtaacgaaagttgcaaaaaatcattcccatatttcctagaaatgttggtttggacaccaggaaaaattctttgaagtggtgaagctaaaaaacaattattaactgtcctctcaatttgattacatccataaattttctctgcagtttgaaatttctgcaattcacccagaccggactgaaaccttaatataagctgattttccatatgcttgttttctacgtccccttgactatgtcgaactctttgaccagtaagattgtttttatgggtcatcggcccttctttataatttatttcaccatctttccattgaaagtcaacttcctgtagatttttccggatttccctgaagtaaaaattttcagtgtcatagctttcatgtccttccaacatcactgcttggaatttttctcctgtgttactgttctgtattggtggtaattccttgatcacacatttaggagagataccggtgatcacgcctttcatgcattccccacagtttgggttcctcgctattttcacttggctcaccacagtccagggctctttcccttgctccaacatggagataatattcaggtcaggaagacagagtcccaggaagccgaggttcctgtagttctccaacatcacgtccctgtacaaagctttctgaacagggtccaggcatttccactcctcctgagagaattctacagccacatccctgaatgtcaaagatccctgaggaagagccatccctggctccttttctttcttctttctctcctgggcctctctctcagtcaatataattaattctttaaaagtcaaatcatagattgaggtgtgcgattcagttgcccgccatttcaagataaattaatctggtgtaaggaccattgggacgaaggggctgttgcgggtattttaaggtccgtagcgatccccaggtcacgggtatggagaaccgaggactgcgaagtgcacgtttaatcaaggtagacgaagagaagcaaacgtttaatccaggtagactgaaacacactcatagcgacgtggcctttccccagcgcgatctgcttccgggtgt

SEQ ID NO: 15839 - RNA, 3251 nt, Homo sapiens
  source 1..3251: mol_type = other RNA
gctgggattacaggcatgagccagacctcatgagaactatcacaaggacagcaacaaggggatggtactaaaactttcttgagaaagccacccccatcatccaatcacctcccactaggctccacctccaatactggagattactacaattccacatgagacttcaaagggaaaggacaaatatacaagctatatgagtaagtataaattatttggggatcccagaggttaggacaacatctaacggcctttccacattgagtttagttgtaaggttctctccagcatgttttatctgatgtttagtgaggcctgagcgactaatgtaagatttgccacactcattacatttataaggtttttcactagaatgaattcgttggtgtttagtgaggcaagaccgccgcccaaacgccttgccacattccatacatttgtatggcttctctccagtatggtttctctgatggtaaaccaagtttgacctttcgataaaagctttaccacattcattacatttataaggtttctctccagtatgcatcatctgatgattaagcagaattgaacgtactctaaaggctttgccacactcattacatttgtaaggtttctctccagtatgaatactccaatgacgtgcgaggcctgagcgataacggaagaccttgccacattcattacatttgtaaggtttctctccagtatgaattctccgatgccttgccagggttgtagtggagttaaagactttcccacattcaatacatttgtatggcatctctccagtatgtcttctctgatggtacaccagacttgttttatgactaaaagttctaccacattcactacatttgtgtggtttctccccagtaggatttctgtgatatcttgcaagttttgaactttggataaaagcctcaccaaattcattacagtggtaagggttctctccagtatgaattaccagatgtttagtgaggcttgaacgctgagtataggctttgccacaatcattacatttataaggtttctctccggtatgaattttccgatgacgtgctaggcatgagtagtaactgaagaccttgccgcattcgttacactggaaaggtttctctccggtatgacttcgcctatgaattgaaaggtttccactgtcaatgaagaccttgccacacacattacatttgtaaggtttctctccggtatgcattctttgatgacgtgctaggcatgaatagtaagtgaagaccatgccacatttattacaatggagaggtttctctccagtatgacatctcatatgaaccgaaaggtatccaccgtaattaaagaccttgccacacacattacatttgtaaggtttctctccggtatgaattctctgatgtacagttagtaatgagccccaattaaaggctttgccacattcattacatttgtaaggtttctctccagtatgaactctctgatgcactgcaagatgtgaatgttgactgaagaccttgccacattcattacatttgtagggtttctctccagtatgaattctccggtgccctgcaagacgtgaacgttgaaagaagaccttgccacattcattacatttgtaaggtgtctctccagtatgaattatctggtgccttacaagttgtgaattctgataaaagaccttgccacatacatcacatgtatatggtttctttcctgcatggattatatgatgtgcagtgaggcttgagttccgtttaaaggttttgccacattcattacatttgtagggtttgtctccagtatgaactgtctgatgagttgcaagagaggaactttgactaaagcacttcccacatcgattacatttgtaaggtttctctccagtatgaattctctgatgaactgcaaggtgggaacttttactaaaggacttgccacattcattacatatgtagggtttgtctccagtgtgacttctccggtgatttacaagatctgaattttgtctgaagatcctgccacatacatcacattggtatggtttccctcttgtatggactatctgatgtactgttagtagtgagccccgatgaaaggctttaccagactcattgcatctgtaaggtttctctgtagtatgtatcatctgatgattaataagacttgaagacactctgaaggctttgccacactcattacctatgtaaggtttttccctaatatgtgttttctcgtcttgtgtaggtaacgaaagttgcaaaaaatcattcccatatttcctagaaatgttggtttggacaccaggaaaaattctttgaagtggtgaagctaaaaaacaattattaactgtcctctcaatttgattacatccataaattttctctgcagtttgaaatttctgcaattcacccagaccggactgaaaccttaatataagctgattttccatatgcttgttttctacgtccccttgactatgtcgaactctttgaccagtaagattgtttttatgggtcatcggcccttctttataatttatttcaccatctttccattgaaagtcaacttcctgtagatttttccggatttccctgaagtaaaaattttcagtgtcatagctttcatgtccttccaacatcactgcttggaatttttctcctgtgttactgttctgtattggtggtaattccttgatcacacatttaggagagataccggtgatcacgcctttcatgcattccccacagtttgggttcctcgctattttcacttggctcaccacagtccagggctctttcccttgctccaacatggagataatattcaggtcaggaagacagagtcccaggaagccgaggttcctgtagttctccaacatcacgtccctgtacaaagctttctgaacagggtccaggcatttccactcctcctgagagaattctacagccacatccctgaatgtcaaagatccctgaggaagagccatccctggctccttttctttcttctttctctcctgggcctctctctcagtcaatataattaattctttaaaagtcaaatttgggacgaaggggctgttgcgggtattttaaggtccgtagcgatccccaggtcacgggtatggagaaccgaggactgcgaagtgcacgtttaatcaaggtagacgaagagaagcaaacgtttaatccaggtagactgaaacacactcatagcgacgtggcctttccccagcgcgatctgcttccgggtgt

SEQ ID NO: 15840 - RNA, 3555 nt, Homo sapiens
  source 1..3555: mol_type = other RNA
gctgggattacaggcatgagccagacctcatgagaactatcacaaggacagcaacaaggggatggtactaaaactttcttgagaaagccacccccatcatccaatcacctcccactaggctccacctccaatactggagattactacaattccacatgagacttcaaagggaaaggacaaatatacaagctatatgagtaagtataaattatttggggatcccagaggttaggacaacatctaacggcctttccacattgagtttagttgtaaggttctctccagcatgttttatctgatgtttagtgaggcctgagcgactaatgtaagatttgccacactcattacatttataaggtttttcactagaatgaattcgttggtgtttagtgaggcaagaccgccgcccaaacgccttgccacattccatacatttgtatggcttctctccagtatggtttctctgatggtaaaccaagtttgacctttcgataaaagctttaccacattcattacatttataaggtttctctccagtatgcatcatctgatgattaagcagaattgaacgtactctaaaggctttgccacactcattacatttgtaaggtttctctccagtatgaatactccaatgacgtgcgaggcctgagcgataacggaagaccttgccacattcattacatttgtaaggtttctctccagtatgaattctccgatgccttgccagggttgtagtggagttaaagactttcccacattcaatacatttgtatggcatctctccagtatgtcttctctgatggtacaccagacttgttttatgactaaaagttctaccacattcactacatttgtgtggtttctccccagtaggatttctgtgatatcttgcaagttttgaactttggataaaagcctcaccaaattcattacagtggtaagggttctctccagtatgaattaccagatgtttagtgaggcttgaacgctgagtataggctttgccacaatcattacatttataaggtttctctccggtatgaattttccgatgacgtgctaggcatgagtagtaactgaagaccttgccgcattcgttacactggaaaggtttctctccggtatgacttcgcctatgaattgaaaggtttccactgtcaatgaagaccttgccacacacattacatttgtaaggtttctctccggtatgcattctttgatgacgtgctaggcatgaatagtaagtgaagaccatgccacatttattacaatggagaggtttctctccagtatgacatctcatatgaaccgaaaggtatccaccgtaattaaagaccttgccacacacattacatttgtaaggtttctctccggtatgaattctctgatgtacagttagtaatgagccccaattaaaggctttgccacattcattacatttgtaaggtttctctccagtatgaactctctgatgcactgcaagatgtgaatgttgactgaagaccttgccacattcattacatttgtagggtttctctccagtatgaattctccggtgccctgcaagacgtgaacgttgaaagaagaccttgccacattcattacatttgtaaggtgtctctccagtatgaattatctggtgccttacaagttgtgaattctgataaaagaccttgccacatacatcacatgtatatggtttctttcctgcatggattatatgatgtgcagtgaggcttgagttccgtttaaaggttttgccacattcattacatttgtagggtttgtctccagtatgaactgtctgatgagttgcaagagaggaactttgactaaagcacttcccacatcgattacatttgtaaggtttctctccagtatgaattctctgatgaactgcaaggtgggaacttttactaaaggacttgccacattcattacatatgtagggtttgtctccagtgtgacttctccggtgatttacaagatctgaattttgtctgaagatcctgccacatacatcacattggtatggtttccctcttgtatggactatctgatgtactgttagtagtgagccccgatgaaaggctttaccagactcattgcatctgtaaggtttctctgtagtatgtatcatctgatgattaataagacttgaagacactctgaaggctttgccacactcattacctatgtaaggtttttccctaatatgtgttttctcgtcttgtgtaggtaacgaaagttgcaaaaaatcattcccatatttcctagaaatgttggtttggacaccaggaaaaattctttgaagtggtgaagctaaaaaacaattattaactgtcctctcaatttgattacatccataaattttctctgcagtttgaaatttctgcaattcacccagaccggactgaaaccttaatataagctgattttccatatgcttgttttctacgtccccttgactatgtcgaactctttgaccagtaagattgtttttatgggtcatcggcccttctttataatttatttcaccatctttccattgaaagtcaacttcctgtagatttttccggatttccctgaagtaaaaattttcagtgtcatagctttcatgtccttccaacatcactgcttggaatttttctcctgtgttactgttctgtattggtggtaattccttgatcacacatttaggagagataccggtgatcacgcctttcatgcattccccacagtttgggttcctcgctattttcacttggctcaccacagtccagggctctttcccttgctccaacatggagataatattcaggtcaggaagacagagtcctgccaggaagccgaggttcctgtagttctccaacatcacgtccctgtacaaagctttctgaacagggtccaggcatttccactcctcctgagagaattctacagccacatccctgaatgtcaaagatccctgaggaagagccatccctggctccttttctttcttctttctctcctgggcctctctctcagtcaatataattaattctttaaaagtcaaatcatagattgaggtgtgcgattcagttgcccgccatttcaagataaattaatctggtgtaaggaccacttgtaggcctagtgtggtggctcacatctgtaattccagtgcgttgagaggctgaggtggaaagactgcttgaggccaggaagtagaagctgcagtgagccgagatcatgccactgctctccagcctaggcggcagagagagaccatgtccccccccaaaacaaaacagaacaaagccaaaaaaaacaccaaagacatatcttgtagtgacagtcagtcatttcttgccccatttctcccctcctttatgctctactccatcattgggaagaagagagttaccacaaataactggatcaagtcactgccctctggctaaataggaattccaaatatcttttgatacaaatacatacaaaatgcacaaggcttatagaaaaaactttggtgattttcatcctcatgagtacaacttaaacatattt

SEQ ID NO: 15841 - RNA, 3401 nt, Homo sapiens
  source 1..3401: mol_type = other RNA
gctgggattacaggcatgagccagacctcatgagaactatcacaaggacagcaacaaggggatggtactaaaactttcttgagaaagccacccccatcatccaatcacctcccactaggctccacctccaatactggagattactacaattccacatgagacttcaaagggaaaggacaaatatacaagctatatgagtaagtataaattatttggggatcccagaggttaggacaacatctaacggcctttccacattgagtttagttgtaaggttctctccagcatgttttatctgatgtttagtgaggcctgagcgactaatgtaagatttgccacactcattacatttataaggtttttcactagaatgaattcgttggtgtttagtgaggcaagaccgccgcccaaacgccttgccacattccatacatttgtatggcttctctccagtatggtttctctgatggtaaaccaagtttgacctttcgataaaagctttaccacattcattacatttataaggtttctctccagtatgcatcatctgatgattaagcagaattgaacgtactctaaaggctttgccacactcattacatttgtaaggtttctctccagtatgaatactccaatgacgtgcgaggcctgagcgataacggaagaccttgccacattcattacatttgtaaggtttctctccagtatgaattctccgatgccttgccagggttgtagtggagttaaagactttcccacattcaatacatttgtatggcatctctccagtatgtcttctctgatggtacaccagacttgttttatgactaaaagttctaccacattcactacatttgtgtggtttctccccagtaggatttctgtgatatcttgcaagttttgaactttggataaaagcctcaccaaattcattacagtggtaagggttctctccagtatgaattaccagatgtttagtgaggcttgaacgctgagtataggctttgccacaatcattacatttataaggtttctctccggtatgaattttccgatgacgtgctaggcatgagtagtaactgaagaccttgccgcattcgttacactggaaaggtttctctccggtatgacttcgcctatgaattgaaaggtttccactgtcaatgaagaccttgccacacacattacatttgtaaggtttctctccggtatgcattctttgatgacgtgctaggcatgaatagtaagtgaagaccatgccacatttattacaatggagaggtttctctccagtatgacatctcatatgaaccgaaaggtatccaccgtaattaaagaccttgccacacacattacatttgtaaggtttctctccggtatgaattctctgatgtacagttagtaatgagccccaattaaaggctttgccacattcattacatttgtaaggtttctctccagtatgaactctctgatgcactgcaagatgtgaatgttgactgaagaccttgccacattcattacatttgtagggtttctctccagtatgaattctccggtgccctgcaagacgtgaacgttgaaagaagaccttgccacattcattacatttgtaaggtgtctctccagtatgaattatctggtgccttacaagttgtgaattctgataaaagaccttgccacatacatcacatgtatatggtttctttcctgcatggattatatgatgtgcagtgaggcttgagttccgtttaaaggttttgccacattcattacatttgtagggtttgtctccagtatgaactgtctgatgagttgcaagagaggaactttgactaaagcacttcccacatcgattacatttgtaaggtttctctccagtatgaattctctgatgaactgcaaggtgggaacttttactaaaggacttgccacattcattacatatgtagggtttgtctccagtgtgacttctccggtgatttacaagatctgaattttgtctgaagatcctgccacatacatcacattggtatggtttccctcttgtatggactatctgatgtactgttagtagtgagccccgatgaaaggctttaccagactcattgcatctgtaaggtttctctgtagtatgtatcatctgatgattaataagacttgaagacactctgaaggctttgccacactcattacctatgtaaggtttttccctaatatgtgttttctcgtcttgtgtaggtaacgaaagttgcaaaaaatcattcccatatttcctagaaatgttggtttggacaccaggaaaaattctttgaagtggtgaagctaaaaaacaattattaactgtcctctcaatttgattacatccataaattttctctgcagtttgaaatttctgcaattcacccagaccggactgaaaccttaatataagctgattttccatatgcttgttttctacgtccccttgactatgtcgaactctttgaccagtaagattgtttttatgggtcatcggcccttctttataatttatttcaccatctttccattgaaagtcaacttcctgtagatttttccggatttccctgaagtaaaaattttcagtgtcatagctttcatgtccttccaacatcactgcttggaatttttctcctgtgttactgttctgtattggtggtaattccttgatcacacatttaggagagataccggtgatcacgcctttcatgcattccccacagtttgggttcctcgctattttcacttggctcaccacagtccagggctctttcccttgctccaacatggagataatattcaggtcaggaagacagagtcctgccaggaagccgaggttcctgtagttctccaacatcacgtccctgtacaaagctttctgaacagggtccaggcatttccactcctcctgagagaattctacagccacatccctgaatgtcaaagatccctgaggaagagccatccctggctccttttctttcttctttctctcctgggcctctctctcagtcaatataattaattctttaaaagtcaaatcatagattgaggtgtgcgattcagttgcccgccatttcaagataaattaatctggtgtaaggaccacttgtaggcctagtgtggtggctcacatctgtaattccagtgcgttgagaggctgaggtggaaagattgggacgaaggggctgttgcgggtattttaaggtccgtagcgatccccaggtcacgggtatggagaaccgaggactgcgaagtgcacgtttaatcaaggtagacgaagagaagcaaacgtttaatccaggtagactgaaacacactcatagcgacgtggcctttccccagcgcgatctgcttccgggtgtgcaggaaactgggcg

SEQ ID NO: 15842 - RNA, 3187 nt, Homo sapiens
  source 1..3187: mol_type = other RNA
gctgggattacaggcatgagccagacctcatgagaactatcacaaggacagcaacaaggggatggtactaaaactttcttgagaaagccacccccatcatccaatcacctcccactaggctccacctccaatactggagattactacaattccacatgagacttcaaagggaaaggacaaatatacaagctatatgagtaagtataaattatttggggatcccagaggttaggacaacatctaacggcctttccacattgagtttagttgtaaggttctctccagcatgttttatctgatgtttagtgaggcctgagcgactaatgtaagatttgccacactcattacatttataaggtttttcactagaatgaattcgttggtgtttagtgaggcaagaccgccgcccaaacgccttgccacattccatacatttgtatggcttctctccagtatggtttctctgatggtaaaccaagtttgacctttcgataaaagctttaccacattcattacatttataaggtttctctccagtatgcatcatctgatgattaagcagaattgaacgtactctaaaggctttgccacactcattacatttgtaaggtttctctccagtatgaatactccaatgacgtgcgaggcctgagcgataacggaagaccttgccacattcattacatttgtaaggtttctctccagtatgaattctccgatgccttgccagggttgtagtggagttaaagactttcccacattcaatacatttgtatggcatctctccagtatgtcttctctgatggtacaccagacttgttttatgactaaaagttctaccacattcactacatttgtgtggtttctccccagtaggatttctgtgatatcttgcaagttttgaactttggataaaagcctcaccaaattcattacagtggtaagggttctctccagtatgaattaccagatgtttagtgaggcttgaacgctgagtataggctttgccacaatcattacatttataaggtttctctccggtatgaattttccgatgacgtgctaggcatgagtagtaactgaagaccttgccgcattcgttacactggaaaggtttctctccggtatgacttcgcctatgaattgaaaggtttccactgtcaatgaagaccttgccacacacattacatttgtaaggtttctctccggtatgcattctttgatgacgtgctaggcatgaatagtaagtgaagaccatgccacatttattacaatggagaggtttctctccagtatgacatctcatatgaaccgaaaggtatccaccgtaattaaagaccttgccacacacattacatttgtaaggtttctctccggtatgaattctctgatgtacagttagtaatgagccccaattaaaggctttgccacattcattacatttgtaaggtttctctccagtatgaactctctgatgcactgcaagatgtgaatgttgactgaagaccttgccacattcattacatttgtagggtttctctccagtatgaattctccggtgccctgcaagacgtgaacgttgaaagaagaccttgccacattcattacatttgtaaggtgtctctccagtatgaattatctggtgccttacaagttgtgaattctgataaaagaccttgccacatacatcacatgtatatggtttctttcctgcatggattatatgatgtgcagtgaggcttgagttccgtttaaaggttttgccacattcattacatttgtagggtttgtctccagtatgaactgtctgatgagttgcaagagaggaactttgactaaagcacttcccacatcgattacatttgtaaggtttctctccagtatgaattctctgatgaactgcaaggtgggaacttttactaaaggacttgccacattcattacatatgtagggtttgtctccagtgtgacttctccggtgatttacaagatctgaattttgtctgaagatcctgccacatacatcacattggtatggtttccctcttgtatggactatctgatgtactgttagtagtgagccccgatgaaaggctttaccagactcattgcatctgtaaggtttctctgtagtatgtatcatctgatgattaataagacttgaagacactctgaaggctttgccacactcattacctatgtaaggtttttccctaatatgtgttttctcgtcttgtgtaggtaacgaaagttgcaaaaaatcattcccatatttcctagaaatgttggtttggacaccaggaaaaattctttgaagtggtgaagctaaaaaacaattattaactgtcctctcaatttgattacatccataaattttctctgcagtttgaaatttctgcaattcacccagaccggactgaaaccttaatataagctgattttccatatgcttgttttctacgtccccttgactatgtcgaactctttgaccagtaagattgtttttatgggtcatcggcccttctttataatttatttcaccatctttccattgaaagtcaacttcctgtagatttttccggatttccctgaagtaaaaattttcagtgtcatagctttcatgtccttccaacatcactgcttggaatttttctcctgtgttactgttctgtattggtggtaattccttgatcacacatttaggagagatacctgaggaagagccatccctggctccttttctttcttctttctctcctgggcctctctctcagtcaatataattaattctttaaaagtcaaatcatagattgaggtgtgcgattcagttgcccgccatttcaagataaattaatctggtgtaaggaccacttgtaggcctagtgtggtggctcacatctgtaattccagtgcgttgagaggctgaggtggaaagactgcttgaggccaggaagtagaagctgcagtgagccgagatcatgccactgctctccagcttgggacgaaggggctgttgcgggtattttaaggtccgtagcgatccccaggtcacgggtatggagaaccgaggactgcgaagtgcacgtttaatcaaggtagacgaagagaagcaaacgtttaatccaggtagactgaaacacactcatagcgacgtggcctttccccagcgcgatctgcttccgggtgt

SEQ ID NO: 15843 - RNA, 3202 nt, Homo sapiens
  source 1..3202: mol_type = other RNA
gctgggattacaggcatgagccagacctcatgagaactatcacaaggacagcaacaaggggatggtactaaaactttcttgagaaagccacccccatcatccaatcacctcccactaggctccacctccaatactggagattactacaattccacatgagacttcaaagggaaaggacaaatatacaagctatatgagtaagtataaattatttggggatcccagaggttaggacaacatctaacggcctttccacattgagtttagttgtaaggttctctccagcatgttttatctgatgtttagtgaggcctgagcgactaatgtaagatttgccacactcattacatttataaggtttttcactagaatgaattcgttggtgtttagtgaggcaagaccgccgcccaaacgccttgccacattccatacatttgtatggcttctctccagtatggtttctctgatggtaaaccaagtttgacctttcgataaaagctttaccacattcattacatttataaggtttctctccagtatgcatcatctgatgattaagcagaattgaacgtactctaaaggctttgccacactcattacatttgtaaggtttctctccagtatgaatactccaatgacgtgcgaggcctgagcgataacggaagaccttgccacattcattacatttgtaaggtttctctccagtatgaattctccgatgccttgccagggttgtagtggagttaaagactttcccacattcaatacatttgtatggcatctctccagtatgtcttctctgatggtacaccagacttgttttatgactaaaagttctaccacattcactacatttgtgtggtttctccccagtaggatttctgtgatatcttgcaagttttgaactttggataaaagcctcaccaaattcattacagtggtaagggttctctccagtatgaattaccagatgtttagtgaggcttgaacgctgagtataggctttgccacaatcattacatttataaggtttctctccggtatgaattttccgatgacgtgctaggcatgagtagtaactgaagaccttgccgcattcgttacactggaaaggtttctctccggtatgacttcgcctatgaattgaaaggtttccactgtcaatgaagaccttgccacacacattacatttgtaaggtttctctccggtatgcattctttgatgacgtgctaggcatgaatagtaagtgaagaccatgccacatttattacaatggagaggtttctctccagtatgacatctcatatgaaccgaaaggtatccaccgtaattaaagaccttgccacacacattacatttgtaaggtttctctccggtatgaattctctgatgtacagttagtaatgagccccaattaaaggctttgccacattcattacatttgtaaggtttctctccagtatgaactctctgatgcactgcaagatgtgaatgttgactgaagaccttgccacattcattacatttgtagggtttctctccagtatgaattctccggtgccctgcaagacgtgaacgttgaaagaagaccttgccacattcattacatttgtaaggtgtctctccagtatgaattatctggtgccttacaagttgtgaattctgataaaagaccttgccacatacatcacatgtatatggtttctttcctgcatggattatatgatgtgcagtgaggcttgagttccgtttaaaggttttgccacattcattacatttgtagggtttgtctccagtatgaactgtctgatgagttgcaagagaggaactttgactaaagcacttcccacatcgattacatttgtaaggtttctctccagtatgaattctctgatgaactgcaaggtgggaacttttactaaaggacttgccacattcattacatatgtagggtttgtctccagtgtgacttctccggtgatttacaagatctgaattttgtctgaagatcctgccacatacatcacattggtatggtttccctcttgtatggactatctgatgtactgttagtagtgagccccgatgaaaggctttaccagactcattgcatctgtaaggtttctctgtagtatgtatcatctgatgattaataagacttgaagacactctgaaggctttgccacactcattacctatgtaaggtttttccctaatatgtgttttctcgtcttgtgtaggtaacgaaagttgcaaaaaatcattcccatatttcctagaaatgttggtttggacaccaggaaaaattctttgaagtggtgaagctaaaaaacaattattaactgtcctctcaatttgattacatccataaattttctctgcagtttgaaatttctgcaattcacccagaccggactgaaaccttaatataagctgattttccatatgcttgttttctacgtccccttgactatgtcgaactctttgaccagtaagattgtttttatgggtcatcggcccttctttataatttatttcaccatctttccattgaaagtcaacttcctgtagatttttccggatttccctgaagtaaaaattttcagtgtcatagctttcatgtccttccaacatcactgcttggaatttttctcctgtgttactgttctgtattggtggtaattccttgatcacacatttaggagagatacctgaggaagagccatccctggctccttttctttcttctttctctcctgggcctctctctcagtcaatataattaattctttaaaagtcaaatcatagattgaggtgtgcgattcagttgcccgccatttcaagataaattaatctggtgtaaggaccacttgtaggcctagtgtggtggctcacatctgtaattccagtgcgttgagaggctgaggtggaaagactgcttgaggccaggaagtagaagctgcagtgagccgagatcatgccactgctctccagcttgggacgaaggggctgttgcgggtattttaaggtccgtagcgatccccaggtcacgggtatggagaaccgaggactgcgaagtgcacgtttaatcaaggtagacgaagagaagcaaacgtttaatccaggtagactgaaacacactcatagcgacgtggcctttccccagcgcgatctgcttccgggtgtgcaggaaactgggcg

SEQ ID NO: 15844 - RNA, 2995 nt, Homo sapiens
  source 1..2995: mol_type = other RNA
gctgggattacaggcatgagccagacctcatgagaactatcacaaggacagcaacaaggggatggtactaaaactttcttgagaaagccacccccatcatccaatcacctcccactaggctccacctccaatactggagattactacaattccacatgagacttcaaagggaaaggacaaatatacaagctatatgagtaagtataaattatttggggatcccagaggttaggacaacatctaacggcctttccacattgagtttagttgtaaggttctctccagcatgttttatctgatgtttagtgaggcctgagcgactaatgtaagatttgccacactcattacatttataaggtttttcactagaatgaattcgttggtgtttagtgaggcaagaccgccgcccaaacgccttgccacattccatacatttgtatggcttctctccagtatggtttctctgatggtaaaccaagtttgacctttcgataaaagctttaccacattcattacatttataaggtttctctccagtatgcatcatctgatgattaagcagaattgaacgtactctaaaggctttgccacactcattacatttgtaaggtttctctccagtatgaatactccaatgacgtgcgaggcctgagcgataacggaagaccttgccacattcattacatttgtaaggtttctctccagtatgaattctccgatgccttgccagggttgtagtggagttaaagactttcccacattcaatacatttgtatggcatctctccagtatgtcttctctgatggtacaccagacttgttttatgactaaaagttctaccacattcactacatttgtgtggtttctccccagtaggatttctgtgatatcttgcaagttttgaactttggataaaagcctcaccaaattcattacagtggtaagggttctctccagtatgaattaccagatgtttagtgaggcttgaacgctgagtataggctttgccacaatcattacatttataaggtttctctccggtatgaattttccgatgacgtgctaggcatgagtagtaactgaagaccttgccgcattcgttacactggaaaggtttctctccggtatgacttcgcctatgaattgaaaggtttccactgtcaatgaagaccttgccacacacattacatttgtaaggtttctctccggtatgcattctttgatgacgtgctaggcatgaatagtaagtgaagaccatgccacatttattacaatggagaggtttctctccagtatgacatctcatatgaaccgaaaggtatccaccgtaattaaagaccttgccacacacattacatttgtaaggtttctctccggtatgaattctctgatgtacagttagtaatgagccccaattaaaggctttgccacattcattacatttgtaaggtttctctccagtatgaactctctgatgcactgcaagatgtgaatgttgactgaagaccttgccacattcattacatttgtagggtttctctccagtatgaattctccggtgccctgcaagacgtgaacgttgaaagaagaccttgccacattcattacatttgtaaggtgtctctccagtatgaattatctggtgccttacaagttgtgaattctgataaaagaccttgccacatacatcacatgtatatggtttctttcctgcatggattatatgatgtgcagtgaggcttgagttccgtttaaaggttttgccacattcattacatttgtagggtttgtctccagtatgaactgtctgatgagttgcaagagaggaactttgactaaagcacttcccacatcgattacatttgtaaggtttctctccagtatgaattctctgatgaactgcaaggtgggaacttttactaaaggacttgccacattcattacatatgtagggtttgtctccagtgtgacttctccggtgatttacaagatctgaattttgtctgaagatcctgccacatacatcacattggtatggtttccctcttgtatggactatctgatgtactgttagtagtgagccccgatgaaaggctttaccagactcattgcatctgtaaggtttctctgtagtatgtatcatctgatgattaataagacttgaagacactctgaaggctttgccacactcattacctatgtaaggtttttccctaatatgtgttttctcgtcttgtgtaggtaacgaaagttgcaaaaaatcattcccatatttcctagaaatgttggtttggacaccaggaaaaattctttgaagtggtgaagctaaaaaacaattattaactgtcctctcaatttgattacatccataaattttctctgcagtttgaaatttctgcaattcacccagaccggactgaaaccttaatataagctgattttccatatgcttgttttctacgtccccttgactatgtcgaactctttgaccagtaagattgtttttatgggtcatcggcccttctttataatttatttcaccatctttccattgaaagtcaacttcctgtagatttttccggatttccctgaagtaaaaattttcagtgtcatagctttcatgtccttccaacatcactgcttggaatttttctcctgtgttactgttctgtattggtggtaattccttgatcacacatttaggagagatacctgaggaagagccatccctggctccttttctttcttctttctctcctgggcctctctctcagtcaatataattaattctttaaaagtcaaatttgggacgaaggggctgttgcgggtattttaaggtccgtagcgatccccaggtcacgggtatggagaaccgaggactgcgaagtgcacgtttaatcaaggtagacgaagagaagcaaacgtttaatccaggtagactgaaacacactcatagcgacgtggcctttccccagcgcgatctgcttccgggtgt

SEQ ID NO: 15845 - RNA, 5729 nt, Homo sapiens
  source 1..5729: mol_type = other RNA
gctgggattacaggcatgagccagagcacctggtctatttttttttttttaaattaagaaacacgttggtcatggtggctcatggctgtaatcccagcaccttgggaggccaatacggctggatcgcttgagccctggaattcaagaccagctcgggcaacatggtgaaagcccatctctactaggaacacaaaaatttgcccggtgcggtggcacctggctatggtcctagcaactttggaggctgaggtgggaggatcccttgaacccaggagattgaagcttcagtgagggctgatcctgtcaccgctctcatgcctggccaacagaatgagacccatctttaatagaaatgaagaaaaaggaaacacatgcgtcctgggtctggggacagggagagtctaaggccaattaacacgaacctcaggaggtcctgatgacgtgtgtccatggtgttgaggctgcagtttggtttcacacattttacagacacacgagacagcaatcagtacatatatacattggtccggtctggaaaggtggaataactggaattggggaccttctgggtcacaggtagataacaaataacattctttgaatctttgatcagcctttcactaaatacacaatttatatgtgagcagggaggagggataagtcacttatgccttaggctggctcagggaccctgtatttttacataaatagggcaagggaagcaatcagatagacatttgactcaggtgtgcagagggatgggctctttcccacatctgtgaagataagctctcagtttacatcgccagggtgaaattcaacagaactattttagggtggagatcttgaggttcccggtttgggaggggcatatgtagctttttaaaaaatctttgtaactatcttgtttaggaataaaatggaaggcaggtttgtctgacgcagttcccagattgacttttctctttggcttagtaatttttattttcctttcacaagcttgtgacagccataatgctttgacacactgatactgttttatatagatttttccacaacagtaaagtccaagggtctgtcatgaaccgggttagagaagatgagaaaattttcagaagactccatctcaaaaaaacaaaacaaacaaaacagaatttaaaatacagaattaagtcatttgactttttttaaatgaaaagtctcacatatttattactgaaccaagccaacaaaggtgttcataacagatccagagaaaaaaaatacattctcaataaaacatgtccaactctccagatagtggtgacattttcagcttgatatggtaacgtgactgaatcttcagacagcatgaatatgtgtgccatctcatatgcaattccttatagatccagcttggctcttctccagtgtcgtctttgacagttgtacctataaaacttatgtggatggtctgcctgccactctgtgcatcactttcttttttttttttttttttttttttttgagatggagtctcgctctgtcacccaggctggagtgcagtagcatgatctctgctcatggcaagctccacctcctcggttcatgccattctcctgcctcagcctcctgagtagctgggactacaggcgcccacaaccacgcctggctaattttttgtatttttagtagagatggggtttcaccgtgttagccaggattttctcgatctcctgacctcgtgatgctcttgcctcggcctcccaaagtgctgggattacaggtgtgagccaccacacctgtcctgtgcatcactttcaacatcatcttgtcccaacttaaaataagttttccatttacaaactggtgatttattttgggaatcgtccccataaccttttcataaagcatcaatgatttcattgtccctctacccaaactttaccagattcatttttcgatacactatctgtctctgtcacccatgctggagtacaatggcatgatcatggctccctgcagcctcgaactcctaggctcaagccatcctcccactgcagactccacagaagctgaaccagcagacatgtgccacaatgcccagctaatttatgtattttttgtagagaaggtggtttcaccattctgcccaggctggtcttgagtaccggggcccacgtgacccaactgtctcagcctctgaaaattatgggattacaggcctgagccacagcatctggtctcatcgcaaatttgatgtttcttcttgtttcagttttagcagaatttacattgccttgattgagtctcttttcaaactcatgtcttacccatctgagtgcctcaaaccaaaccctgttcagacatgttataacggatttgtatcagtttatcttggtgcaaaaaatgtgatatcatgcacaattttctcataatatgtatttttccatgaacttcctgaagaccccttgtactagcgaactgtattcaagaggttataaaaaggattgttgatatgcaagtgccacttatttctgggatgcaaaatggttcaacatagtcaagcaaatcaatgtgatataccacttgaacataatgaaagatgaaaaccacatcatctcaatacatggagaaaaagcatttcacaaaattcaacatccagtcatcatggaaatcctaaacaaaatagaaagagaaggaaatttacctcaacaatacaaagaccatccatgaaatgaccacagcagaaataaccagtcagggaaaatggaatgcttttcctgtaggatctcacatgatgcaagaatgctctcaccccttctattcaatcaatactggctgtcctagctagagcaatgaaatagcaaaagaaatcaaactcatccaaatcagaaagaaagaagtaaaactatttctttgtagatgacatgatcttctgtgtagaaaatcacaaagagtcaaccaaaatgcaactggaactaaaaaacatatgcagtggatttgaagaatagaataacagcaccaaaaattagttgaatttccatacattaacaataaacaatttaaaaagaaaattaaaaaaacactttcatttgctaaagaacttaaagtaagaaatacttaggaataaatgaaaaaagttgagaagtttctaccttcaaatctacaaacattgatcaaagtgataaaaacatgtgcaaataagagatacaagccatattgaatggaataatattgctaaatgattataactgaatgtgatgtagattcaacacaatacccagagaaatttctataactttttgttaaagaaacaaaaaacaggccaggtgtggtggctcacgcctgtaatctcagcactttggcaggtggaggcaggtggattttaaggacagaagatcgagaccatcctagctaacacggtgaaacccagtctctactaaaaatacaaaaaattacccgggcatggtggcacgcacctgtagtcccagctactcaggagactgaggcaggagaattgcatgaacctgggaggtgaatgttgcagtgaaccgagatcacatcactgcactccaacgtgggcgacagagcaagattccatcttaaaaataaataaataaataaaagaacatacaggctgggaaaagtggctcccgtctgttggccaggctggtctcaaattcatgacctcaagtgacctacctgtcttggcctctcaaagtgctgggattacaggtgtgagacaccacgcctggcccaatcctcttaacataaacagtttaatgtcgattaatgcttgaaatcaatgttaagtcaactcaaactcaggtcaatgctgatttgactctgatgtcaattaatgcttgatggtttgctatactcattgcacttgaaacaattgtctccaaaaggaattttctgatgttctgcaaggagtgacctcagactaaagaccttgccacactgatgacatttgtaagatttctgtccagtatggattctctgatgcctaataaggtgtgaaggtgaattaaaggctttaccacaatcaccacacttgtgaggtttctctcctgtatgaatcctcctatgtctttcaaggtgtgatttgcgaatgtaaactttgtcacattcttcacattcgtaaagtttctctccagtatgaagtttttgatgacatgcgaggtacgcttttgtactaaaaaccttgccacattcattacatgtgtaaggtctctctccagtatgaactctctgatgttctgcaagacgtgaatcactccggaaagccttgtcacaaaccttacatttgtatggtttctctccagtatgaatcctcctatgtctttcaagatgtgatttgcgactgaaaactttgtcgcattcttcacatctgtaaggtttctctccagtgtgaactctacgatgtcctgcaagagttgctcgttgcttaaaaaccttgccacattcattacacttatagggtttctctgcagtatgaactgccttatgaattacgaggactgaatttcgagcgaaggtcttgccacactcattacatttgtaaggtttctctccagtatgcagtctatgatggtacacaaggtgtgatgtctgactaaaggtcttgccacactcattacacttataaggtttctctccagtatgacttctatgatgacatgcaagggttgctttttgatcaaaaaccttgccacattcattacatgtgtaatgtttgtctcccctgtgaattctagtatgttttgccaggtgtgaatcatgcttaaaagccttgtcgcaaaccttacatttgtatggtttctctccagtatgaattatcctatgtatttcaagatgtgatttgcaactgaaaactttctcacattcttcacatttgtaaggtttctctccagtatgaattctcctatgtcttcgcaaatgcaaatgaaatcttgattcaagctgacctttaataggcttgtttccagcatgcctttgatcatatcggtctgtactactagtcaacttttttatttctgtcatgggtgcttcatggtcatttgtttcatcttcttgccactgaaacacaaagtcatgaatgtctttctcaatttcctgggagcaaaatgctccaatgtgataacttgcttgtctctgcaatgtccctgtgtggatcacttctgtattgccttgccctgttgatgacaatgtattcatcatgcatttggaagagatatccagggagaccaggttcctataattctccagcatcacgtctctgtatagagtcctctgagcagggtccaggcatttccactcctcctgagagaattctatggccacatccctgaatgtcagtagaccctgagaaagagccatccccgactcctttgctttcctcttcctcttctgggtttcttcctcaggtaccaagagtctttagaagtcaatcctgtatctcagctacttggtaggctgaggcacaagaatcacttgaacccaggagacagaggttgcagtgagccaagatcaggagactgcactcacagccaggctgaggtgggagaattgcttgagcccggagagcagaggttgaagtgaatcaagatcgcacaactgccctccagcccggacgtctcaatttgctctgggttgagaaagaggggccgcaatttccaggtctgtggggactcaacgtccccggtatagcagcaccacaggactgggaagcacacataaaacag

SEQ ID NO: 15846 - RNA, 5749 nt, Homo sapiens
  source 1..5749: mol_type = other RNA
gctgggattacaggcatgagccagagcacctggtctatttttttttttttaaattaagaaacacgttggtcatggtggctcatggctgtaatcccagcaccttgggaggccaatacggctggatcgcttgagccctggaattcaagaccagctcgggcaacatggtgaaagcccatctctactaggaacacaaaaatttgcccggtgcggtggcacctggctatggtcctagcaactttggaggctgaggtgggaggatcccttgaacccaggagattgaagcttcagtgagggctgatcctgtcaccgctctcatgcctggccaacagaatgagacccatctttaatagaaatgaagaaaaaggaaacacatgcgtcctgggtctggggacagggagagtctaaggccaattaacacgaacctcaggaggtcctgatgacgtgtgtccatggtgttgaggctgcagtttggtttcacacattttacagacacacgagacagcaatcagtacatatatacattggtccggtctggaaaggtggaataactggaattggggaccttctgggtcacaggtagataacaaataacattctttgaatctttgatcagcctttcactaaatacacaatttatatgtgagcagggaggagggataagtcacttatgccttaggctggctcagggaccctgtatttttacataaatagggcaagggaagcaatcagatagacatttgactcaggtgtgcagagggatgggctctttcccacatctgtgaagataagctctcagtttacatcgccagggtgaaattcaacagaactattttagggtggagatcttgaggttcccggtttgggaggggcatatgtagctttttaaaaaatctttgtaactatcttgtttaggaataaaatggaaggcaggtttgtctgacgcagttcccagattgacttttctctttggcttagtaatttttattttcctttcacaagcttgtgacagccataatgctttgacacactgatactgttttatatagatttttccacaacagtaaagtccaagggtctgtcatgaaccgggttagagaagatgagaaaattttcagaagactccatctcaaaaaaacaaaacaaacaaaacagaatttaaaatacagaattaagtcatttgactttttttaaatgaaaagtctcacatatttattactgaaccaagccaacaaaggtgttcataacagatccagagaaaaaaaatacattctcaataaaacatgtccaactctccagatagtggtgacattttcagcttgatatggtaacgtgactgaatcttcagacagcatgaatatgtgtgccatctcatatgcaattccttatagatccagcttggctcttctccagtgtcgtctttgacagttgtacctataaaacttatgtggatggtctgcctgccactctgtgcatcactttcttttttttttttttttttttttttttgagatggagtctcgctctgtcacccaggctggagtgcagtagcatgatctctgctcatggcaagctccacctcctcggttcatgccattctcctgcctcagcctcctgagtagctgggactacaggcgcccacaaccacgcctggctaattttttgtatttttagtagagatggggtttcaccgtgttagccaggattttctcgatctcctgacctcgtgatgctcttgcctcggcctcccaaagtgctgggattacaggtgtgagccaccacacctgtcctgtgcatcactttcaacatcatcttgtcccaacttaaaataagttttccatttacaaactggtgatttattttgggaatcgtccccataaccttttcataaagcatcaatgatttcattgtccctctacccaaactttaccagattcatttttcgatacactatctgtctctgtcacccatgctggagtacaatggcatgatcatggctccctgcagcctcgaactcctaggctcaagccatcctcccactgcagactccacagaagctgaaccagcagacatgtgccacaatgcccagctaatttatgtattttttgtagagaaggtggtttcaccattctgcccaggctggtcttgagtaccggggcccacgtgacccaactgtctcagcctctgaaaattatgggattacaggcctgagccacagcatctggtctcatcgcaaatttgatgtttcttcttgtttcagttttagcagaatttacattgccttgattgagtctcttttcaaactcatgtcttacccatctgagtgcctcaaaccaaaccctgttcagacatgttataacggatttgtatcagtttatcttggtgcaaaaaatgtgatatcatgcacaattttctcataatatgtatttttccatgaacttcctgaagaccccttgtactagcgaactgtattcaagaggttataaaaaggattgttgatatgcaagtgccacttatttctgggatgcaaaatggttcaacatagtcaagcaaatcaatgtgatataccacttgaacataatgaaagatgaaaaccacatcatctcaatacatggagaaaaagcatttcacaaaattcaacatccagtcatcatggaaatcctaaacaaaatagaaagagaaggaaatttacctcaacaatacaaagaccatccatgaaatgaccacagcagaaataaccagtcagggaaaatggaatgcttttcctgtaggatctcacatgatgcaagaatgctctcaccccttctattcaatcaatactggctgtcctagctagagcaatgaaatagcaaaagaaatcaaactcatccaaatcagaaagaaagaagtaaaactatttctttgtagatgacatgatcttctgtgtagaaaatcacaaagagtcaaccaaaatgcaactggaactaaaaaacatatgcagtggatttgaagaatagaataacagcaccaaaaattagttgaatttccatacattaacaataaacaatttaaaaagaaaattaaaaaaacactttcatttgctaaagaacttaaagtaagaaatacttaggaataaatgaaaaaagttgagaagtttctaccttcaaatctacaaacattgatcaaagtgataaaaacatgtgcaaataagagatacaagccatattgaatggaataatattgctaaatgattataactgaatgtgatgtagattcaacacaatacccagagaaatttctataactttttgttaaagaaacaaaaaacaggccaggtgtggtggctcacgcctgtaatctcagcactttggcaggtggaggcaggtggattttaaggacagaagatcgagaccatcctagctaacacggtgaaacccagtctctactaaaaatacaaaaaattacccgggcatggtggcacgcacctgtagtcccagctactcaggagactgaggcaggagaattgcatgaacctgggaggtgaatgttgcagtgaaccgagatcacatcactgcactccaacgtgggcgacagagcaagattccatcttaaaaataaataaataaataaaagaacatacaggctgggaaaagtggctcccgtctgttggccaggctggtctcaaattcatgacctcaagtgacctacctgtcttggcctctcaaagtgctgggattacaggtgtgagacaccacgcctggcccaatcctcttaacataaacagtttaatgtcgattaatgcttgaaatcaatgttaagtcaactcaaactcaggtcaatgctgatttgactctgatgtcaattaatgcttgatggtttgctatactcattgcacttgaaacaattgtctccaaaaggaattttctgatgttctgcaaggagtgacctcagactaaagaccttgccacactgatgacatttgtaagatttctgtccagtatggattctctgatgcctaataaggtgtgaaggtgaattaaaggctttaccacaatcaccacacttgtgaggtttctctcctgtatgaatcctcctatgtctttcaaggtgtgatttgcgaatgtaaactttgtcacattcttcacattcgtaaagtttctctccagtatgaagtttttgatgacatgcgaggtacgcttttgtactaaaaaccttgccacattcattacatgtgtaaggtctctctccagtatgaactctctgatgttctgcaagacgtgaatcactccggaaagccttgtcacaaaccttacatttgtatggtttctctccagtatgaatcctcctatgtctttcaagatgtgatttgcgactgaaaactttgtcgcattcttcacatctgtaaggtttctctccagtgtgaactctacgatgtcctgcaagagttgctcgttgcttaaaaaccttgccacattcattacacttatagggtttctctgcagtatgaactgccttatgaattacgaggactgaatttcgagcgaaggtcttgccacactcattacatttgtaaggtttctctccagtatgcagtctatgatggtacacaaggtgtgatgtctgactaaaggtcttgccacactcattacacttataaggtttctctccagtatgacttctatgatgacatgcaagggttgctttttgatcaaaaaccttgccacattcattacatgtgtaatgtttgtctcccctgtgaattctagtatgttttgccaggtgtgaatcatgcttaaaagccttgtcgcaaaccttacatttgtatggtttctctccagtatgaattatcctatgtatttcaagatgtgatttgcaactgaaaactttctcacattcttcacatttgtaaggtttctctccagtatgaattctcctatgtcttcgcaaatgcaaatgaaatcttgattcaagctgacctttaataggcttgtttccagcatgcctttgatcatatcggtctgtactactagtcaacttttttatttctgtcatgggtgcttcatggtcatttgtttcatcttcttgccactgaaacacaaagtcatgaatgtctttctcaatttcctgggagcaaaatgctccaatgtgataacttgcttgtctctgcaatgtccctgtgtggatcacttctgtattgccttgccctgttgatgacaatgtattcatcatgcatttggaagagatatccagggagaccaggttcctataattctccagcatcacgtctctgtatagagtcctctgagcagggtccaggcatttccactcctcctgagagaattctatggccacatccctgaatgtcagtagaccctgagaaagagccatccccgactcctttgctttcctcttcctcttctgggtttcttcctcaggtaccaagagtctttagaagtcaatcctgtatctcagctacttggtaggctgaggcacaagaatcacttgaacccaggagacagaggttgcagtgagccaagatcaggagactgcactcacagcctgaaggacagagtgagactcaggctgaggtgggagaattgcttgagcccggagagcagaggttgaagtgaatcaagatcgcacaactgccctccagcccggacgtctcaatttgctctgggttgagaaagaggggccgcaatttccaggtctgtggggactcaacgtccccggtatagcagcaccacaggactgggaagcacacataaaacag

SEQ ID NO: 15847 - RNA, 5791 nt, Homo sapiens
  source 1..5791: mol_type = other RNA
gctgggattacaggcatgagccagagcacctggtctatttttttttttttaaattaagaaacacgttggtcatggtggctcatggctgtaatcccagcaccttgggaggccaatacggctggatcgcttgagccctggaattcaagaccagctcgggcaacatggtgaaagcccatctctactaggaacacaaaaatttgcccggtgcggtggcacctggctatggtcctagcaactttggaggctgaggtgggaggatcccttgaacccaggagattgaagcttcagtgagggctgatcctgtcaccgctctcatgcctggccaacagaatgagacccatctttaatagaaatgaagaaaaaggaaacacatgcgtcctgggtctggggacagggagagtctaaggccaattaacacgaacctcaggaggtcctgatgacgtgtgtccatggtgttgaggctgcagtttggtttcacacattttacagacacacgagacagcaatcagtacatatatacattggtccggtctggaaaggtggaataactggaattggggaccttctgggtcacaggtagataacaaataacattctttgaatctttgatcagcctttcactaaatacacaatttatatgtgagcagggaggagggataagtcacttatgccttaggctggctcagggaccctgtatttttacataaatagggcaagggaagcaatcagatagacatttgactcaggtgtgcagagggatgggctctttcccacatctgtgaagataagctctcagtttacatcgccagggtgaaattcaacagaactattttagggtggagatcttgaggttcccggtttgggaggggcatatgtagctttttaaaaaatctttgtaactatcttgtttaggaataaaatggaaggcaggtttgtctgacgcagttcccagattgacttttctctttggcttagtaatttttattttcctttcacaagcttgtgacagccataatgctttgacacactgatactgttttatatagatttttccacaacagtaaagtccaagggtctgtcatgaaccgggttagagaagatgagaaaattttcagaagactccatctcaaaaaaacaaaacaaacaaaacagaatttaaaatacagaattaagtcatttgactttttttaaatgaaaagtctcacatatttattactgaaccaagccaacaaaggtgttcataacagatccagagaaaaaaaatacattctcaataaaacatgtccaactctccagatagtggtgacattttcagcttgatatggtaacgtgactgaatcttcagacagcatgaatatgtgtgccatctcatatgcaattccttatagatccagcttggctcttctccagtgtcgtctttgacagttgtacctataaaacttatgtggatggtctgcctgccactctgtgcatcactttcttttttttttttttttttttttttttgagatggagtctcgctctgtcacccaggctggagtgcagtagcatgatctctgctcatggcaagctccacctcctcggttcatgccattctcctgcctcagcctcctgagtagctgggactacaggcgcccacaaccacgcctggctaattttttgtatttttagtagagatggggtttcaccgtgttagccaggattttctcgatctcctgacctcgtgatgctcttgcctcggcctcccaaagtgctgggattacaggtgtgagccaccacacctgtcctgtgcatcactttcaacatcatcttgtcccaacttaaaataagttttccatttacaaactggtgatttattttgggaatcgtccccataaccttttcataaagcatcaatgatttcattgtccctctacccaaactttaccagattcatttttcgatacactatctgtctctgtcacccatgctggagtacaatggcatgatcatggctccctgcagcctcgaactcctaggctcaagccatcctcccactgcagactccacagaagctgaaccagcagacatgtgccacaatgcccagctaatttatgtattttttgtagagaaggtggtttcaccattctgcccaggctggtcttgagtaccggggcccacgtgacccaactgtctcagcctctgaaaattatgggattacaggcctgagccacagcatctggtctcatcgcaaatttgatgtttcttcttgtttcagttttagcagaatttacattgccttgattgagtctcttttcaaactcatgtcttacccatctgagtgcctcaaaccaaaccctgttcagacatgttataacggatttgtatcagtttatcttggtgcaaaaaatgtgatatcatgcacaattttctcataatatgtatttttccatgaacttcctgaagaccccttgtactagcgaactgtattcaagaggttataaaaaggattgttgatatgcaagtgccacttatttctgggatgcaaaatggttcaacatagtcaagcaaatcaatgtgatataccacttgaacataatgaaagatgaaaaccacatcatctcaatacatggagaaaaagcatttcacaaaattcaacatccagtcatcatggaaatcctaaacaaaatagaaagagaaggaaatttacctcaacaatacaaagaccatccatgaaatgaccacagcagaaataaccagtcagggaaaatggaatgcttttcctgtaggatctcacatgatgcaagaatgctctcaccccttctattcaatcaatactggctgtcctagctagagcaatgaaatagcaaaagaaatcaaactcatccaaatcagaaagaaagaagtaaaactatttctttgtagatgacatgatcttctgtgtagaaaatcacaaagagtcaaccaaaatgcaactggaactaaaaaacatatgcagtggatttgaagaatagaataacagcaccaaaaattagttgaatttccatacattaacaataaacaatttaaaaagaaaattaaaaaaacactttcatttgctaaagaacttaaagtaagaaatacttaggaataaatgaaaaaagttgagaagtttctaccttcaaatctacaaacattgatcaaagtgataaaaacatgtgcaaataagagatacaagccatattgaatggaataatattgctaaatgattataactgaatgtgatgtagattcaacacaatacccagagaaatttctataactttttgttaaagaaacaaaaaacaggccaggtgtggtggctcacgcctgtaatctcagcactttggcaggtggaggcaggtggattttaaggacagaagatcgagaccatcctagctaacacggtgaaacccagtctctactaaaaatacaaaaaattacccgggcatggtggcacgcacctgtagtcccagctactcaggagactgaggcaggagaattgcatgaacctgggaggtgaatgttgcagtgaaccgagatcacatcactgcactccaacgtgggcgacagagcaagattccatcttaaaaataaataaataaataaaagaacatacaggctgggaaaagtggctcccgtctgttggccaggctggtctcaaattcatgacctcaagtgacctacctgtcttggcctctcaaagtgctgggattacaggtgtgagacaccacgcctggcccaatcctcttaacataaacagtttaatgtcgattaatgcttgaaatcaatgttaagtcaactcaaactcaggtcaatgctgatttgactctgatgtcaattaatgcttgatggtttgctatactcattgcacttgaaacaattgtctccaaaaggaattttctgatgttctgcaaggagtgacctcagactaaagaccttgccacactgatgacatttgtaagatttctgtccagtatggattctctgatgcctaataaggtgtgaaggtgaattaaaggctttaccacaatcaccacacttgtgaggtttctctcctgtatgaatcctcctatgtctttcaaggtgtgatttgcgaatgtaaactttgtcacattcttcacattcgtaaagtttctctccagtatgaagtttttgatgacatgcgaggtacgcttttgtactaaaaaccttgccacattcattacatgtgtaaggtctctctccagtatgaactctctgatgttctgcaagacgtgaatcactccggaaagccttgtcacaaaccttacatttgtatggtttctctccagtatgaatcctcctatgtctttcaagatgtgatttgcgactgaaaactttgtcgcattcttcacatctgtaaggtttctctccagtgtgaactctacgatgtcctgcaagagttgctcgttgcttaaaaaccttgccacattcattacacttatagggtttctctgcagtatgaactgccttatgaattacgaggactgaatttcgagcgaaggtcttgccacactcattacatttgtaaggtttctctccagtatgcagtctatgatggtacacaaggtgtgatgtctgactaaaggtcttgccacactcattacacttataaggtttctctccagtatgacttctatgatgacatgcaagggttgctttttgatcaaaaaccttgccacattcattacatgtgtaatgtttgtctcccctgtgaattctagtatgttttgccaggtgtgaatcatgcttaaaagccttgtcgcaaaccttacatttgtatggtttctctccagtatgaattatcctatgtatttcaagatgtgatttgcaactgaaaactttctcacattcttcacatttgtaaggtttctctccagtatgaattctcctatgtcttcgcaaatgcaaatgaaatcttgattcaagctgacctttaataggcttgtttccagcatgcctttgatcatatcggtctgtactactagtcaacttttttatttctgtcatgggtgcttcatggtcatttgtttcatcttcttgccactgaaacacaaagtcatgaatgtctttctcaatttcctgggagcaaaatgctccaatgtgataacttgcttgtctctgcaatgtccctgtgtggatcacttctgtattgccttgccctgttgatgacaatgtattcatcatgcatttggaagagatatccagggagaccaggttcctataattctccagcatcacgtctctgtatagagtcctctgagcagggtccaggcatttccactcctcctgagagaattctatggccacatccctgaatgtcagtagaccctgagaaagagccatccccgactcctttgctttcctcttcctcttctgggtttcttcctcaggtaccaagagtctttagaagtcaatcctgtatctcagctacttggtaggctgaggcacaagaatcacttgaacccaggagacagaggttgcagtgagccaagatcaggagactgcactcacagcctgaaggacagagtgagactcaggctgaggtgggagaattgcttgagcccggagagcagaggttgaagtgaatcaagatcgcacaactgccctccagcctcagggccactttaaactcgaagggactcacggactctcacccggacgtctcaatttgctctgggttgagaaagaggggccgcaatttccaggtctgtggggactcaacgtccccggtatagcagcaccacaggactgggaagcacacataaaacag

SEQ ID NO: 15848 - RNA, 5820 nt, Homo sapiens
  source 1..5820: mol_type = other RNA
gctgggattacaggcatgagccagagcacctggtctatttttttttttttaaattaagaaacacgttggtcatggtggctcatggctgtaatcccagcaccttgggaggccaatacggctggatcgcttgagccctggaattcaagaccagctcgggcaacatggtgaaagcccatctctactaggaacacaaaaatttgcccggtgcggtggcacctggctatggtcctagcaactttggaggctgaggtgggaggatcccttgaacccaggagattgaagcttcagtgagggctgatcctgtcaccgctctcatgcctggccaacagaatgagacccatctttaatagaaatgaagaaaaaggaaacacatgcgtcctgggtctggggacagggagagtctaaggccaattaacacgaacctcaggaggtcctgatgacgtgtgtccatggtgttgaggctgcagtttggtttcacacattttacagacacacgagacagcaatcagtacatatatacattggtccggtctggaaaggtggaataactggaattggggaccttctgggtcacaggtagataacaaataacattctttgaatctttgatcagcctttcactaaatacacaatttatatgtgagcagggaggagggataagtcacttatgccttaggctggctcagggaccctgtatttttacataaatagggcaagggaagcaatcagatagacatttgactcaggtgtgcagagggatgggctctttcccacatctgtgaagataagctctcagtttacatcgccagggtgaaattcaacagaactattttagggtggagatcttgaggttcccggtttgggaggggcatatgtagctttttaaaaaatctttgtaactatcttgtttaggaataaaatggaaggcaggtttgtctgacgcagttcccagattgacttttctctttggcttagtaatttttattttcctttcacaagcttgtgacagccataatgctttgacacactgatactgttttatatagatttttccacaacagtaaagtccaagggtctgtcatgaaccgggttagagaagatgagaaaattttcagaagactccatctcaaaaaaacaaaacaaacaaaacagaatttaaaatacagaattaagtcatttgactttttttaaatgaaaagtctcacatatttattactgaaccaagccaacaaaggtgttcataacagatccagagaaaaaaaatacattctcaataaaacatgtccaactctccagatagtggtgacattttcagcttgatatggtaacgtgactgaatcttcagacagcatgaatatgtgtgccatctcatatgcaattccttatagatccagcttggctcttctccagtgtcgtctttgacagttgtacctataaaacttatgtggatggtctgcctgccactctgtgcatcactttcttttttttttttttttttttttttttgagatggagtctcgctctgtcacccaggctggagtgcagtagcatgatctctgctcatggcaagctccacctcctcggttcatgccattctcctgcctcagcctcctgagtagctgggactacaggcgcccacaaccacgcctggctaattttttgtatttttagtagagatggggtttcaccgtgttagccaggattttctcgatctcctgacctcgtgatgctcttgcctcggcctcccaaagtgctgggattacaggtgtgagccaccacacctgtcctgtgcatcactttcaacatcatcttgtcccaacttaaaataagttttccatttacaaactggtgatttattttgggaatcgtccccataaccttttcataaagcatcaatgatttcattgtccctctacccaaactttaccagattcatttttcgatacactatctgtctctgtcacccatgctggagtacaatggcatgatcatggctccctgcagcctcgaactcctaggctcaagccatcctcccactgcagactccacagaagctgaaccagcagacatgtgccacaatgcccagctaatttatgtattttttgtagagaaggtggtttcaccattctgcccaggctggtcttgagtaccggggcccacgtgacccaactgtctcagcctctgaaaattatgggattacaggcctgagccacagcatctggtctcatcgcaaatttgatgtttcttcttgtttcagttttagcagaatttacattgccttgattgagtctcttttcaaactcatgtcttacccatctgagtgcctcaaaccaaaccctgttcagacatgttataacggatttgtatcagtttatcttggtgcaaaaaatgtgatatcatgcacaattttctcataatatgtatttttccatgaacttcctgaagaccccttgtactagcgaactgtattcaagaggttataaaaaggattgttgatatgcaagtgccacttatttctgggatgcaaaatggttcaacatagtcaagcaaatcaatgtgatataccacttgaacataatgaaagatgaaaaccacatcatctcaatacatggagaaaaagcatttcacaaaattcaacatccagtcatcatggaaatcctaaacaaaatagaaagagaaggaaatttacctcaacaatacaaagaccatccatgaaatgaccacagcagaaataaccagtcagggaaaatggaatgcttttcctgtaggatctcacatgatgcaagaatgctctcaccccttctattcaatcaatactggctgtcctagctagagcaatgaaatagcaaaagaaatcaaactcatccaaatcagaaagaaagaagtaaaactatttctttgtagatgacatgatcttctgtgtagaaaatcacaaagagtcaaccaaaatgcaactggaactaaaaaacatatgcagtggatttgaagaatagaataacagcaccaaaaattagttgaatttccatacattaacaataaacaatttaaaaagaaaattaaaaaaacactttcatttgctaaagaacttaaagtaagaaatacttaggaataaatgaaaaaagttgagaagtttctaccttcaaatctacaaacattgatcaaagtgataaaaacatgtgcaaataagagatacaagccatattgaatggaataatattgctaaatgattataactgaatgtgatgtagattcaacacaatacccagagaaatttctataactttttgttaaagaaacaaaaaacaggccaggtgtggtggctcacgcctgtaatctcagcactttggcaggtggaggcaggtggattttaaggacagaagatcgagaccatcctagctaacacggtgaaacccagtctctactaaaaatacaaaaaattacccgggcatggtggcacgcacctgtagtcccagctactcaggagactgaggcaggagaattgcatgaacctgggaggtgaatgttgcagtgaaccgagatcacatcactgcactccaacgtgggcgacagagcaagattccatcttaaaaataaataaataaataaaagaacatacaggctgggaaaagtggctcccgtctgttggccaggctggtctcaaattcatgacctcaagtgacctacctgtcttggcctctcaaagtgctgggattacaggtgtgagacaccacgcctggcccaatcctcttaacataaacagtttaatgtcgattaatgcttgaaatcaatgttaagtcaactcaaactcaggtcaatgctgatttgactctgatgtcaattaatgcttgatggtttgctatactcattgcacttgaaacaattgtctccaaaaggaattttctgatgttctgcaaggagtgacctcagactaaagaccttgccacactgatgacatttgtaagatttctgtccagtatggattctctgatgcctaataaggtgtgaaggtgaattaaaggctttaccacaatcaccacacttgtgaggtttctctcctgtatgaatcctcctatgtctttcaaggtgtgatttgcgaatgtaaactttgtcacattcttcacattcgtaaagtttctctccagtatgaagtttttgatgacatgcgaggtacgcttttgtactaaaaaccttgccacattcattacatgtgtaaggtctctctccagtatgaactctctgatgttctgcaagacgtgaatcactccggaaagccttgtcacaaaccttacatttgtatggtttctctccagtatgaatcctcctatgtctttcaagatgtgatttgcgactgaaaactttgtcgcattcttcacatctgtaaggtttctctccagtgtgaactctacgatgtcctgcaagagttgctcgttgcttaaaaaccttgccacattcattacacttatagggtttctctgcagtatgaactgccttatgaattacgaggactgaatttcgagcgaaggtcttgccacactcattacatttgtaaggtttctctccagtatgcagtctatgatggtacacaaggtgtgatgtctgactaaaggtcttgccacactcattacacttataaggtttctctccagtatgacttctatgatgacatgcaagggttgctttttgatcaaaaaccttgccacattcattacatgtgtaatgtttgtctcccctgtgaattctagtatgttttgccaggtgtgaatcatgcttaaaagccttgtcgcaaaccttacatttgtatggtttctctccagtatgaattatcctatgtatttcaagatgtgatttgcaactgaaaactttctcacattcttcacatttgtaaggtttctctccagtatgaattctcctatgtcttcgcaaatgcaaatgaaatcttgattcaagctgacctttaataggcttgtttccagcatgcctttgatcatatcggtctgtactactagtcaacttttttatttctgtcatgggtgcttcatggtcatttgtttcatcttcttgccactgaaacacaaagtcatgaatgtctttctcaatttcctgggagcaaaatgctccaatgtgataacttgcttgtctctgcaatgtccctgtgtggatcacttctgtattgccttgccctgttgatgacaatgtattcatcatgcatttggaagagatatccagggagaccaggttcctataattctccagcatcacgtctctgtatagagtcctctgagcagggtccaggcatttccactcctcctgagagaattctatggccacatccctgaatgtcagtagaccctgagaaagagccatccccgactcctttgctttcctcttcctcttctgggtttcttcctcaggtaccaagagtctttagaagtcaatcctgtatctcagctacttggtaggctgaggcacaagaatcacttgaacccaggagacagaggttgcagtgagccaagatcaggagactgcactcacagcctgaaggacagagtgagactcaggctgaggtgggagaattgcttgagcccggagagcagaggttgaagtgaatcaagatcgcacaactgccctccagcctgggggacacagcgaaactccatcacctccaccccccaaaaagttggaagctcactgaattaagatacaaccggacgtctcaatttgctctgggttgagaaagaggggccgcaatttccaggtctgtggggactcaacgtccccggtatagcagcaccacaggactgggaagcacacataaaacag

SEQ ID NO: 15849 - RNA, 5941 nt, Homo sapiens
  source 1..5941: mol_type = other RNA
gctgggattacaggcatgagccagagcacctggtctatttttttttttttaaattaagaaacacgttggtcatggtggctcatggctgtaatcccagcaccttgggaggccaatacggctggatcgcttgagccctggaattcaagaccagctcgggcaacatggtgaaagcccatctctactaggaacacaaaaatttgcccggtgcggtggcacctggctatggtcctagcaactttggaggctgaggtgggaggatcccttgaacccaggagattgaagcttcagtgagggctgatcctgtcaccgctctcatgcctggccaacagaatgagacccatctttaatagaaatgaagaaaaaggaaacacatgcgtcctgggtctggggacagggagagtctaaggccaattaacacgaacctcaggaggtcctgatgacgtgtgtccatggtgttgaggctgcagtttggtttcacacattttacagacacacgagacagcaatcagtacatatatacattggtccggtctggaaaggtggaataactggaattggggaccttctgggtcacaggtagataacaaataacattctttgaatctttgatcagcctttcactaaatacacaatttatatgtgagcagggaggagggataagtcacttatgccttaggctggctcagggaccctgtatttttacataaatagggcaagggaagcaatcagatagacatttgactcaggtgtgcagagggatgggctctttcccacatctgtgaagataagctctcagtttacatcgccagggtgaaattcaacagaactattttagggtggagatcttgaggttcccggtttgggaggggcatatgtagctttttaaaaaatctttgtaactatcttgtttaggaataaaatggaaggcaggtttgtctgacgcagttcccagattgacttttctctttggcttagtaatttttattttcctttcacaagcttgtgacagccataatgctttgacacactgatactgttttatatagatttttccacaacagtaaagtccaagggtctgtcatgaaccgggttagagaagatgagaaaattttcagaagactccatctcaaaaaaacaaaacaaacaaaacagaatttaaaatacagaattaagtcatttgactttttttaaatgaaaagtctcacatatttattactgaaccaagccaacaaaggtgttcataacagatccagagaaaaaaaatacattctcaataaaacatgtccaactctccagatagtggtgacattttcagcttgatatggtaacgtgactgaatcttcagacagcatgaatatgtgtgccatctcatatgcaattccttatagatccagcttggctcttctccagtgtcgtctttgacagttgtacctataaaacttatgtggatggtctgcctgccactctgtgcatcactttcttttttttttttttttttttttttttgagatggagtctcgctctgtcacccaggctggagtgcagtagcatgatctctgctcatggcaagctccacctcctcggttcatgccattctcctgcctcagcctcctgagtagctgggactacaggcgcccacaaccacgcctggctaattttttgtatttttagtagagatggggtttcaccgtgttagccaggattttctcgatctcctgacctcgtgatgctcttgcctcggcctcccaaagtgctgggattacaggtgtgagccaccacacctgtcctgtgcatcactttcaacatcatcttgtcccaacttaaaataagttttccatttacaaactggtgatttattttgggaatcgtccccataaccttttcataaagcatcaatgatttcattgtccctctacccaaactttaccagattcatttttcgatacactatctgtctctgtcacccatgctggagtacaatggcatgatcatggctccctgcagcctcgaactcctaggctcaagccatcctcccactgcagactccacagaagctgaaccagcagacatgtgccacaatgcccagctaatttatgtattttttgtagagaaggtggtttcaccattctgcccaggctggtcttgagtaccggggcccacgtgacccaactgtctcagcctctgaaaattatgggattacaggcctgagccacagcatctggtctcatcgcaaatttgatgtttcttcttgtttcagttttagcagaatttacattgccttgattgagtctcttttcaaactcatgtcttacccatctgagtgcctcaaaccaaaccctgttcagacatgttataacggatttgtatcagtttatcttggtgcaaaaaatgtgatatcatgcacaattttctcataatatgtatttttccatgaacttcctgaagaccccttgtactagcgaactgtattcaagaggttataaaaaggattgttgatatgcaagtgccacttatttctgggatgcaaaatggttcaacatagtcaagcaaatcaatgtgatataccacttgaacataatgaaagatgaaaaccacatcatctcaatacatggagaaaaagcatttcacaaaattcaacatccagtcatcatggaaatcctaaacaaaatagaaagagaaggaaatttacctcaacaatacaaagaccatccatgaaatgaccacagcagaaataaccagtcagggaaaatggaatgcttttcctgtaggatctcacatgatgcaagaatgctctcaccccttctattcaatcaatactggctgtcctagctagagcaatgaaatagcaaaagaaatcaaactcatccaaatcagaaagaaagaagtaaaactatttctttgtagatgacatgatcttctgtgtagaaaatcacaaagagtcaaccaaaatgcaactggaactaaaaaacatatgcagtggatttgaagaatagaataacagcaccaaaaattagttgaatttccatacattaacaataaacaatttaaaaagaaaattaaaaaaacactttcatttgctaaagaacttaaagtaagaaatacttaggaataaatgaaaaaagttgagaagtttctaccttcaaatctacaaacattgatcaaagtgataaaaacatgtgcaaataagagatacaagccatattgaatggaataatattgctaaatgattataactgaatgtgatgtagattcaacacaatacccagagaaatttctataactttttgttaaagaaacaaaaaacaggccaggtgtggtggctcacgcctgtaatctcagcactttggcaggtggaggcaggtggattttaaggacagaagatcgagaccatcctagctaacacggtgaaacccagtctctactaaaaatacaaaaaattacccgggcatggtggcacgcacctgtagtcccagctactcaggagactgaggcaggagaattgcatgaacctgggaggtgaatgttgcagtgaaccgagatcacatcactgcactccaacgtgggcgacagagcaagattccatcttaaaaataaataaataaataaaagaacatacaggctgggaaaagtggctcccgtctgttggccaggctggtctcaaattcatgacctcaagtgacctacctgtcttggcctctcaaagtgctgggattacaggtgtgagacaccacgcctggcccaatcctcttaacataaacagtttaatgtcgattaatgcttgaaatcaatgttaagtcaactcaaactcaggtcaatgctgatttgactctgatgtcaattaatgcttgatggtttgctatactcattgcacttgaaacaattgtctccaaaaggaattttctgatgttctgcaaggagtgacctcagactaaagaccttgccacactgatgacatttgtaagatttctgtccagtatggattctctgatgcctaataaggtgtgaaggtgaattaaaggctttaccacaatcaccacacttgtgaggtttctctcctgtatgaatcctcctatgtctttcaaggtgtgatttgcgaatgtaaactttgtcacattcttcacattcgtaaagtttctctccagtatgaagtttttgatgacatgcgaggtacgcttttgtactaaaaaccttgccacattcattacatgtgtaaggtctctctccagtatgaactctctgatgttctgcaagacgtgaatcactccggaaagccttgtcacaaaccttacatttgtatggtttctctccagtatgaatcctcctatgtctttcaagatgtgatttgcgactgaaaactttgtcgcattcttcacatctgtaaggtttctctccagtgtgaactctacgatgtcctgcaagagttgctcgttgcttaaaaaccttgccacattcattacacttatagggtttctctgcagtatgaactgccttatgaattacgaggactgaatttcgagcgaaggtcttgccacactcattacatttgtaaggtttctctccagtatgcagtctatgatggtacacaaggtgtgatgtctgactaaaggtcttgccacactcattacacttataaggtttctctccagtatgacttctatgatgacatgcaagggttgctttttgatcaaaaaccttgccacattcattacatgtgtaatgtttgtctcccctgtgaattctagtatgttttgccaggtgtgaatcatgcttaaaagccttgtcgcaaaccttacatttgtatggtttctctccagtatgaattatcctatgtatttcaagatgtgatttgcaactgaaaactttctcacattcttcacatttgtaaggtttctctccagtatgaattctcctatgtcttcgcaaatgcaaatgaaatcttgattcaagctgacctttaataggcttgtttccagcatgcctttgatcatatcggtctgtactactagtcaacttttttatttctgtcatgggtgcttcatggtcatttgtttcatcttcttgccactgaaacacaaagtcatgaatgtctttctcaatttcctgggagcaaaatgctccaatgtgataacttgcttgtctctgcaatgtccctgtgtggatcacttctgtattgccttgccctgttgatgacaatgtattcatcatgcatttggaagagatatccagggagaccaggttcctataattctccagcatcacgtctctgtatagagtcctctgagcagggtccaggcatttccactcctcctgagagaattctatggccacatccctgaatgtcagtagaccctgagaaagagccatccccgactcctttgctttcctcttcctcttctgggtttcttcctcaggtaccaagagtctttagaagtcaatcctgtatctcagctacttggtaggctgaggcacaagaatcacttgaacccaggagacagaggttgcagtgagccaagatcaggagactgcactcacagcctgaaggacagagtgagactcaggctgaggtgggagaattgcttgagcccggagagcagaggttgaagtgaatcaagatcgcacaactgccctccagcctgtaatcccaggactctgggaggccgaggtgggtggatcacttgaggtcgagttcagagaacagtctggccaatatggtgaaaccttgtctctactgtaatcccggctactggggaggctgaggcaggagatcacttgaacccaggaggcggaggttgtggtgagccaagatcgcgccattgcactccagcccggacgtctcaatttgctctgggttgagaaagaggggccgcaatttccaggtctgtggggactcaacgtccccggtatagcagcaccacaggactgggaagcacacataaaacag

SEQ ID NO: 15850 - RNA, 5759 nt, Homo sapiens
  source 1..5759: mol_type = other RNA
gctgggattacaggcatgagccagagcacctggtctatttttttttttttaaattaagaaacacgttggtcatggtggctcatggctgtaatcccagcaccttgggaggccaatacggctggatcgcttgagccctggaattcaagaccagctcgggcaacatggtgaaagcccatctctactaggaacacaaaaatttgcccggtgcggtggcacctggctatggtcctagcaactttggaggctgaggtgggaggatcccttgaacccaggagattgaagcttcagtgagggctgatcctgtcaccgctctcatgcctggccaacagaatgagacccatctttaatagaaatgaagaaaaaggaaacacatgcgtcctgggtctggggacagggagagtctaaggccaattaacacgaacctcaggaggtcctgatgacgtgtgtccatggtgttgaggctgcagtttggtttcacacattttacagacacacgagacagcaatcagtacatatatacattggtccggtctggaaaggtggaataactggaattggggaccttctgggtcacaggtagataacaaataacattctttgaatctttgatcagcctttcactaaatacacaatttatatgtgagcagggaggagggataagtcacttatgccttaggctggctcagggaccctgtatttttacataaatagggcaagggaagcaatcagatagacatttgactcaggtgtgcagagggatgggctctttcccacatctgtgaagataagctctcagtttacatcgccagggtgaaattcaacagaactattttagggtggagatcttgaggttcccggtttgggaggggcatatgtagctttttaaaaaatctttgtaactatcttgtttaggaataaaatggaaggcaggtttgtctgacgcagttcccagattgacttttctctttggcttagtaatttttattttcctttcacaagcttgtgacagccataatgctttgacacactgatactgttttatatagatttttccacaacagtaaagtccaagggtctgtcatgaaccgggttagagaagatgagaaaattttcagaagactccatctcaaaaaaacaaaacaaacaaaacagaatttaaaatacagaattaagtcatttgactttttttaaatgaaaagtctcacatatttattactgaaccaagccaacaaaggtgttcataacagatccagagaaaaaaaatacattctcaataaaacatgtccaactctccagatagtggtgacattttcagcttgatatggtaacgtgactgaatcttcagacagcatgaatatgtgtgccatctcatatgcaattccttatagatccagcttggctcttctccagtgtcgtctttgacagttgtacctataaaacttatgtggatggtctgcctgccactctgtgcatcactttcttttttttttttttttttttttttttgagatggagtctcgctctgtcacccaggctggagtgcagtagcatgatctctgctcatggcaagctccacctcctcggttcatgccattctcctgcctcagcctcctgagtagctgggactacaggcgcccacaaccacgcctggctaattttttgtatttttagtagagatggggtttcaccgtgttagccaggattttctcgatctcctgacctcgtgatgctcttgcctcggcctcccaaagtgctgggattacaggtgtgagccaccacacctgtcctgtgcatcactttcaacatcatcttgtcccaacttaaaataagttttccatttacaaactggtgatttattttgggaatcgtccccataaccttttcataaagcatcaatgatttcattgtccctctacccaaactttaccagattcatttttcgatacactatctgtctctgtcacccatgctggagtacaatggcatgatcatggctccctgcagcctcgaactcctaggctcaagccatcctcccactgcagactccacagaagctgaaccagcagacatgtgccacaatgcccagctaatttatgtattttttgtagagaaggtggtttcaccattctgcccaggctggtcttgagtaccggggcccacgtgacccaactgtctcagcctctgaaaattatgggattacaggcctgagccacagcatctggtctcatcgcaaatttgatgtttcttcttgtttcagttttagcagaatttacattgccttgattgagtctcttttcaaactcatgtcttacccatctgagtgcctcaaaccaaaccctgttcagacatgttataacggatttgtatcagtttatcttggtgcaaaaaatgtgatatcatgcacaattttctcataatatgtatttttccatgaacttcctgaagaccccttgtactagcgaactgtattcaagaggttataaaaaggattgttgatatgcaagtgccacttatttctgggatgcaaaatggttcaacatagtcaagcaaatcaatgtgatataccacttgaacataatgaaagatgaaaaccacatcatctcaatacatggagaaaaagcatttcacaaaattcaacatccagtcatcatggaaatcctaaacaaaatagaaagagaaggaaatttacctcaacaatacaaagaccatccatgaaatgaccacagcagaaataaccagtcagggaaaatggaatgcttttcctgtaggatctcacatgatgcaagaatgctctcaccccttctattcaatcaatactggctgtcctagctagagcaatgaaatagcaaaagaaatcaaactcatccaaatcagaaagaaagaagtaaaactatttctttgtagatgacatgatcttctgtgtagaaaatcacaaagagtcaaccaaaatgcaactggaactaaaaaacatatgcagtggatttgaagaatagaataacagcaccaaaaattagttgaatttccatacattaacaataaacaatttaaaaagaaaattaaaaaaacactttcatttgctaaagaacttaaagtaagaaatacttaggaataaatgaaaaaagttgagaagtttctaccttcaaatctacaaacattgatcaaagtgataaaaacatgtgcaaataagagatacaagccatattgaatggaataatattgctaaatgattataactgaatgtgatgtagattcaacacaatacccagagaaatttctataactttttgttaaagaaacaaaaaacaggccaggtgtggtggctcacgcctgtaatctcagcactttggcaggtggaggcaggtggattttaaggacagaagatcgagaccatcctagctaacacggtgaaacccagtctctactaaaaatacaaaaaattacccgggcatggtggcacgcacctgtagtcccagctactcaggagactgaggcaggagaattgcatgaacctgggaggtgaatgttgcagtgaaccgagatcacatcactgcactccaacgtgggcgacagagcaagattccatcttaaaaataaataaataaataaaagaacatacaggctgggaaaagtggctcccgtctgttggccaggctggtctcaaattcatgacctcaagtgacctacctgtcttggcctctcaaagtgctgggattacaggtgtgagacaccacgcctggcccaatcctcttaacataaacagtttaatgtcgattaatgcttgaaatcaatgttaagtcaactcaaactcaggtcaatgctgatttgactctgatgtcaattaatgcttgatggtttgctatactcattgcacttgaaacaattgtctccaaaaggaattttctgatgttctgcaaggagtgacctcagactaaagaccttgccacactgatgacatttgtaagatttctgtccagtatggattctctgatgcctaataaggtgtgaaggtgaattaaaggctttaccacaatcaccacacttgtgaggtttctctcctgtatgaatcctcctatgtctttcaaggtgtgatttgcgaatgtaaactttgtcacattcttcacattcgtaaagtttctctccagtatgaagtttttgatgacatgcgaggtacgcttttgtactaaaaaccttgccacattcattacatgtgtaaggtctctctccagtatgaactctctgatgttctgcaagacgtgaatcactccggaaagccttgtcacaaaccttacatttgtatggtttctctccagtatgaatcctcctatgtctttcaagatgtgatttgcgactgaaaactttgtcgcattcttcacatctgtaaggtttctctccagtgtgaactctacgatgtcctgcaagagttgctcgttgcttaaaaaccttgccacattcattacacttatagggtttctctgcagtatgaactgccttatgaattacgaggactgaatttcgagcgaaggtcttgccacactcattacatttgtaaggtttctctccagtatgcagtctatgatggtacacaaggtgtgatgtctgactaaaggtcttgccacactcattacacttataaggtttctctccagtatgacttctatgatgacatgcaagggttgctttttgatcaaaaaccttgccacattcattacatgtgtaatgtttgtctcccctgtgaattctagtatgttttgccaggtgtgaatcatgcttaaaagccttgtcgcaaaccttacatttgtatggtttctctccagtatgaattatcctatgtatttcaagatgtgatttgcaactgaaaactttctcacattcttcacatttgtaaggtttctctccagtatgaattctcctatgtcttcgcaaatgcaaatgaaatcttgattcaagctgacctttaataggcttgtttccagcatgcctttgatcatatcggtctgtactactagtcaacttttttatttctgtcatgggtgcttcatggtcatttgtttcatcttcttgccactgaaacacaaagtcatgaatgtctttctcaatttcctgggagcaaaatgctccaatgtgataacttgcttgtctctgcaatgtccctgtgtggatcacttctgtattgccttgccctgttgatgacaatgtattcatcatgcatttggaagagatatccagggagaccaggttcctataattctccagcatcacgtctctgtatagagtcctctgagcagggtccaggcatttccactcctcctgagagaattctatggccacatccctgaatgtcagtagaccctgagaaagagccatccccgactcctttgctttcctcttcctcttctgggtttcttcctcaggtaccaagagtctttagaagtcaatcctgtatctcagctacttggtaggctgaggcacaagaatcacttgaacccaggagacagaggttgcagtgagccaagatcaggagactgcactcacagcctgaaggacagagtgagactcaggctgaggtgggagaattgcttgagcccggagagcagaggttgaagtgaatcaagatcgcacaactgccctccagcggactctcacccggacgtctcaatttgctctgggttgagaaagaggggccgcaatttccaggtctgtggggactcaacgtccccggtatagcagcaccacaggactgggaagcacacataaaacag

SEQ ID NO: 15851 - RNA, 5671 nt, Homo sapiens
  source 1..5671: mol_type = other RNA
gctgggattacaggcatgagccagagcacctggtctatttttttttttttaaattaagaaacacgttggtcatggtggctcatggctgtaatcccagcaccttgggaggccaatacggctggatcgcttgagccctggaattcaagaccagctcgggcaacatggtgaaagcccatctctactaggaacacaaaaatttgcccggtgcggtggcacctggctatggtcctagcaactttggaggctgaggtgggaggatcccttgaacccaggagattgaagcttcagtgagggctgatcctgtcaccgctctcatgcctggccaacagaatgagacccatctttaatagaaatgaagaaaaaggaaacacatgcgtcctgggtctggggacagggagagtctaaggccaattaacacgaacctcaggaggtcctgatgacgtgtgtccatggtgttgaggctgcagtttggtttcacacattttacagacacacgagacagcaatcagtacatatatacattggtccggtctggaaaggtggaataactggaattggggaccttctgggtcacaggtagataacaaataacattctttgaatctttgatcagcctttcactaaatacacaatttatatgtgagcagggaggagggataagtcacttatgccttaggctggctcagggaccctgtatttttacataaatagggcaagggaagcaatcagatagacatttgactcaggtgtgcagagggatgggctctttcccacatctgtgaagataagctctcagtttacatcgccagggtgaaattcaacagaactattttagggtggagatcttgaggttcccggtttgggaggggcatatgtagctttttaaaaaatctttgtaactatcttgtttaggaataaaatggaaggcaggtttgtctgacgcagttcccagattgacttttctctttggcttagtaatttttattttcctttcacaagcttgtgacagccataatgctttgacacactgatactgttttatatagatttttccacaacagtaaagtccaagggtctgtcatgaaccgggttagagaagatgagaaaattttcagaagactccatctcaaaaaaacaaaacaaacaaaacagaatttaaaatacagaattaagtcatttgactttttttaaatgaaaagtctcacatatttattactgaaccaagccaacaaaggtgttcataacagatccagagaaaaaaaatacattctcaataaaacatgtccaactctccagatagtggtgacattttcagcttgatatggtaacgtgactgaatcttcagacagcatgaatatgtgtgccatctcatatgcaattccttatagatccagcttggctcttctccagtgtcgtctttgacagttgtacctataaaacttatgtggatggtctgcctgccactctgtgcatcactttcttttttttttttttttttttttttttgagatggagtctcgctctgtcacccaggctggagtgcagtagcatgatctctgctcatggcaagctccacctcctcggttcatgccattctcctgcctcagcctcctgagtagctgggactacaggcgcccacaaccacgcctggctaattttttgtatttttagtagagatggggtttcaccgtgttagccaggattttctcgatctcctgacctcgtgatgctcttgcctcggcctcccaaagtgctgggattacaggtgtgagccaccacacctgtcctgtgcatcactttcaacatcatcttgtcccaacttaaaataagttttccatttacaaactggtgatttattttgggaatcgtccccataaccttttcataaagcatcaatgatttcattgtccctctacccaaactttaccagattcatttttcgatacactatctgtctctgtcacccatgctggagtacaatggcatgatcatggctccctgcagcctcgaactcctaggctcaagccatcctcccactgcagactccacagaagctgaaccagcagacatgtgccacaatgcccagctaatttatgtattttttgtagagaaggtggtttcaccattctgcccaggctggtcttgagtaccggggcccacgtgacccaactgtctcagcctctgaaaattatgggattacaggcctgagccacagcatctggtctcatcgcaaatttgatgtttcttcttgtttcagttttagcagaatttacattgccttgattgagtctcttttcaaactcatgtcttacccatctgagtgcctcaaaccaaaccctgttcagacatgttataacggatttgtatcagtttatcttggtgcaaaaaatgtgatatcatgcacaattttctcataatatgtatttttccatgaacttcctgaagaccccttgtactagcgaactgtattcaagaggttataaaaaggattgttgatatgcaagtgccacttatttctgggatgcaaaatggttcaacatagtcaagcaaatcaatgtgatataccacttgaacataatgaaagatgaaaaccacatcatctcaatacatggagaaaaagcatttcacaaaattcaacatccagtcatcatggaaatcctaaacaaaatagaaagagaaggaaatttacctcaacaatacaaagaccatccatgaaatgaccacagcagaaataaccagtcagggaaaatggaatgcttttcctgtaggatctcacatgatgcaagaatgctctcaccccttctattcaatcaatactggctgtcctagctagagcaatgaaatagcaaaagaaatcaaactcatccaaatcagaaagaaagaagtaaaactatttctttgtagatgacatgatcttctgtgtagaaaatcacaaagagtcaaccaaaatgcaactggaactaaaaaacatatgcagtggatttgaagaatagaataacagcaccaaaaattagttgaatttccatacattaacaataaacaatttaaaaagaaaattaaaaaaacactttcatttgctaaagaacttaaagtaagaaatacttaggaataaatgaaaaaagttgagaagtttctaccttcaaatctacaaacattgatcaaagtgataaaaacatgtgcaaataagagatacaagccatattgaatggaataatattgctaaatgattataactgaatgtgatgtagattcaacacaatacccagagaaatttctataactttttgttaaagaaacaaaaaacaggccaggtgtggtggctcacgcctgtaatctcagcactttggcaggtggaggcaggtggattttaaggacagaagatcgagaccatcctagctaacacggtgaaacccagtctctactaaaaatacaaaaaattacccgggcatggtggcacgcacctgtagtcccagctactcaggagactgaggcaggagaattgcatgaacctgggaggtgaatgttgcagtgaaccgagatcacatcactgcactccaacgtgggcgacagagcaagattccatcttaaaaataaataaataaataaaagaacatacaggctgggaaaagtggctcccgtctgttggccaggctggtctcaaattcatgacctcaagtgacctacctgtcttggcctctcaaagtgctgggattacaggtgtgagacaccacgcctggcccaatcctcttaacataaacagtttaatgtcgattaatgcttgaaatcaatgttaagtcaactcaaactcaggtcaatgctgatttgactctgatgtcaattaatgcttgatggtttgctatactcattgcacttgaaacaattgtctccaaaaggaattttctgatgttctgcaaggagtgacctcagactaaagaccttgccacactgatgacatttgtaagatttctgtccagtatggattctctgatgcctaataaggtgtgaaggtgaattaaaggctttaccacaatcaccacacttgtgaggtttctctcctgtatgaatcctcctatgtctttcaaggtgtgatttgcgaatgtaaactttgtcacattcttcacattcgtaaagtttctctccagtatgaagtttttgatgacatgcgaggtacgcttttgtactaaaaaccttgccacattcattacatgtgtaaggtctctctccagtatgaactctctgatgttctgcaagacgtgaatcactccggaaagccttgtcacaaaccttacatttgtatggtttctctccagtatgaatcctcctatgtctttcaagatgtgatttgcgactgaaaactttgtcgcattcttcacatctgtaaggtttctctccagtgtgaactctacgatgtcctgcaagagttgctcgttgcttaaaaaccttgccacattcattacacttatagggtttctctgcagtatgaactgccttatgaattacgaggactgaatttcgagcgaaggtcttgccacactcattacatttgtaaggtttctctccagtatgcagtctatgatggtacacaaggtgtgatgtctgactaaaggtcttgccacactcattacacttataaggtttctctccagtatgacttctatgatgacatgcaagggttgctttttgatcaaaaaccttgccacattcattacatgtgtaatgtttgtctcccctgtgaattctagtatgttttgccaggtgtgaatcatgcttaaaagccttgtcgcaaaccttacatttgtatggtttctctccagtatgaattatcctatgtatttcaagatgtgatttgcaactgaaaactttctcacattcttcacatttgtaaggtttctctccagtatgaattctcctatgtcttcgcaaatgcaaatgaaatcttgattcaagctgacctttaataggcttgtttccagcatgcctttgatcatatcggtctgtactactagtcaacttttttatttctgtcatgggtgcttcatggtcatttgtttcatcttcttgccactgaaacacaaagtcatgaatgtctttctcaatttcctgggagcaaaatgctccaatgtgataacttgcttgtctctgcaatgtccctgtgtggatcacttctgtattgccttgccctgttgatgacaatgtattcatcatgcatttggaagagatatccagggagaccaggttcctataattctccagcatcacgtctctgtatagagtcctctgagcagggtccaggcatttccactcctcctgagagaattctatggccacatccctgaatgtcagtagaccctgagaaagagccatccccgactcctttgctttcctcttcctcttctgggtttcttcctcaggtaccaagagtctttagaagtcaatcctgtatctcagctacttggtaggctgaggcacaagaatcacttgaacccaggagacagaggttgcagtgagccaagatcaggagactgcactcacagcctgaaggacagagtgagactccggacgtctcaatttgctctgggttgagaaagaggggccgcaatttccaggtctgtggggactcaacgtccccggtatagcagcaccacaggactgggaagcacacataaaacag

SEQ ID NO: 15852 - RNA, 5713 nt, Homo sapiens
  source 1..5713: mol_type = other RNA
gctgggattacaggcatgagccagagcacctggtctatttttttttttttaaattaagaaacacgttggtcatggtggctcatggctgtaatcccagcaccttgggaggccaatacggctggatcgcttgagccctggaattcaagaccagctcgggcaacatggtgaaagcccatctctactaggaacacaaaaatttgcccggtgcggtggcacctggctatggtcctagcaactttggaggctgaggtgggaggatcccttgaacccaggagattgaagcttcagtgagggctgatcctgtcaccgctctcatgcctggccaacagaatgagacccatctttaatagaaatgaagaaaaaggaaacacatgcgtcctgggtctggggacagggagagtctaaggccaattaacacgaacctcaggaggtcctgatgacgtgtgtccatggtgttgaggctgcagtttggtttcacacattttacagacacacgagacagcaatcagtacatatatacattggtccggtctggaaaggtggaataactggaattggggaccttctgggtcacaggtagataacaaataacattctttgaatctttgatcagcctttcactaaatacacaatttatatgtgagcagggaggagggataagtcacttatgccttaggctggctcagggaccctgtatttttacataaatagggcaagggaagcaatcagatagacatttgactcaggtgtgcagagggatgggctctttcccacatctgtgaagataagctctcagtttacatcgccagggtgaaattcaacagaactattttagggtggagatcttgaggttcccggtttgggaggggcatatgtagctttttaaaaaatctttgtaactatcttgtttaggaataaaatggaaggcaggtttgtctgacgcagttcccagattgacttttctctttggcttagtaatttttattttcctttcacaagcttgtgacagccataatgctttgacacactgatactgttttatatagatttttccacaacagtaaagtccaagggtctgtcatgaaccgggttagagaagatgagaaaattttcagaagactccatctcaaaaaaacaaaacaaacaaaacagaatttaaaatacagaattaagtcatttgactttttttaaatgaaaagtctcacatatttattactgaaccaagccaacaaaggtgttcataacagatccagagaaaaaaaatacattctcaataaaacatgtccaactctccagatagtggtgacattttcagcttgatatggtaacgtgactgaatcttcagacagcatgaatatgtgtgccatctcatatgcaattccttatagatccagcttggctcttctccagtgtcgtctttgacagttgtacctataaaacttatgtggatggtctgcctgccactctgtgcatcactttcttttttttttttttttttttttttttgagatggagtctcgctctgtcacccaggctggagtgcagtagcatgatctctgctcatggcaagctccacctcctcggttcatgccattctcctgcctcagcctcctgagtagctgggactacaggcgcccacaaccacgcctggctaattttttgtatttttagtagagatggggtttcaccgtgttagccaggattttctcgatctcctgacctcgtgatgctcttgcctcggcctcccaaagtgctgggattacaggtgtgagccaccacacctgtcctgtgcatcactttcaacatcatcttgtcccaacttaaaataagttttccatttacaaactggtgatttattttgggaatcgtccccataaccttttcataaagcatcaatgatttcattgtccctctacccaaactttaccagattcatttttcgatacactatctgtctctgtcacccatgctggagtacaatggcatgatcatggctccctgcagcctcgaactcctaggctcaagccatcctcccactgcagactccacagaagctgaaccagcagacatgtgccacaatgcccagctaatttatgtattttttgtagagaaggtggtttcaccattctgcccaggctggtcttgagtaccggggcccacgtgacccaactgtctcagcctctgaaaattatgggattacaggcctgagccacagcatctggtctcatcgcaaatttgatgtttcttcttgtttcagttttagcagaatttacattgccttgattgagtctcttttcaaactcatgtcttacccatctgagtgcctcaaaccaaaccctgttcagacatgttataacggatttgtatcagtttatcttggtgcaaaaaatgtgatatcatgcacaattttctcataatatgtatttttccatgaacttcctgaagaccccttgtactagcgaactgtattcaagaggttataaaaaggattgttgatatgcaagtgccacttatttctgggatgcaaaatggttcaacatagtcaagcaaatcaatgtgatataccacttgaacataatgaaagatgaaaaccacatcatctcaatacatggagaaaaagcatttcacaaaattcaacatccagtcatcatggaaatcctaaacaaaatagaaagagaaggaaatttacctcaacaatacaaagaccatccatgaaatgaccacagcagaaataaccagtcagggaaaatggaatgcttttcctgtaggatctcacatgatgcaagaatgctctcaccccttctattcaatcaatactggctgtcctagctagagcaatgaaatagcaaaagaaatcaaactcatccaaatcagaaagaaagaagtaaaactatttctttgtagatgacatgatcttctgtgtagaaaatcacaaagagtcaaccaaaatgcaactggaactaaaaaacatatgcagtggatttgaagaatagaataacagcaccaaaaattagttgaatttccatacattaacaataaacaatttaaaaagaaaattaaaaaaacactttcatttgctaaagaacttaaagtaagaaatacttaggaataaatgaaaaaagttgagaagtttctaccttcaaatctacaaacattgatcaaagtgataaaaacatgtgcaaataagagatacaagccatattgaatggaataatattgctaaatgattataactgaatgtgatgtagattcaacacaatacccagagaaatttctataactttttgttaaagaaacaaaaaacaggccaggtgtggtggctcacgcctgtaatctcagcactttggcaggtggaggcaggtggattttaaggacagaagatcgagaccatcctagctaacacggtgaaacccagtctctactaaaaatacaaaaaattacccgggcatggtggcacgcacctgtagtcccagctactcaggagactgaggcaggagaattgcatgaacctgggaggtgaatgttgcagtgaaccgagatcacatcactgcactccaacgtgggcgacagagcaagattccatcttaaaaataaataaataaataaaagaacatacaggctgggaaaagtggctcccgtctgttggccaggctggtctcaaattcatgacctcaagtgacctacctgtcttggcctctcaaagtgctgggattacaggtgtgagacaccacgcctggcccaatcctcttaacataaacagtttaatgtcgattaatgcttgaaatcaatgttaagtcaactcaaactcaggtcaatgctgatttgactctgatgtcaattaatgcttgatggtttgctatactcattgcacttgaaacaattgtctccaaaaggaattttctgatgttctgcaaggagtgacctcagactaaagaccttgccacactgatgacatttgtaagatttctgtccagtatggattctctgatgcctaataaggtgtgaaggtgaattaaaggctttaccacaatcaccacacttgtgaggtttctctcctgtatgaatcctcctatgtctttcaaggtgtgatttgcgaatgtaaactttgtcacattcttcacattcgtaaagtttctctccagtatgaagtttttgatgacatgcgaggtacgcttttgtactaaaaaccttgccacattcattacatgtgtaaggtctctctccagtatgaactctctgatgttctgcaagacgtgaatcactccggaaagccttgtcacaaaccttacatttgtatggtttctctccagtatgaatcctcctatgtctttcaagatgtgatttgcgactgaaaactttgtcgcattcttcacatctgtaaggtttctctccagtgtgaactctacgatgtcctgcaagagttgctcgttgcttaaaaaccttgccacattcattacacttatagggtttctctgcagtatgaactgccttatgaattacgaggactgaatttcgagcgaaggtcttgccacactcattacatttgtaaggtttctctccagtatgcagtctatgatggtacacaaggtgtgatgtctgactaaaggtcttgccacactcattacacttataaggtttctctccagtatgacttctatgatgacatgcaagggttgctttttgatcaaaaaccttgccacattcattacatgtgtaatgtttgtctcccctgtgaattctagtatgttttgccaggtgtgaatcatgcttaaaagccttgtcgcaaaccttacatttgtatggtttctctccagtatgaattatcctatgtatttcaagatgtgatttgcaactgaaaactttctcacattcttcacatttgtaaggtttctctccagtatgaattctcctatgtcttcgcaaatgcaaatgaaatcttgattcaagctgacctttaataggcttgtttccagcatgcctttgatcatatcggtctgtactactagtcaacttttttatttctgtcatgggtgcttcatggtcatttgtttcatcttcttgccactgaaacacaaagtcatgaatgtctttctcaatttcctgggagcaaaatgctccaatgtgataacttgcttgtctctgcaatgtccctgtgtggatcacttctgtattgccttgccctgttgatgacaatgtattcatcatgcatttggaagagatatccagggagaccaggttcctataattctccagcatcacgtctctgtatagagtcctctgagcagggtccaggcatttccactcctcctgagagaattctatggccacatccctgaatgtcagtagaccctgagaaagagccatccccgactcctttgctttcctcttcctcttctgggtttcttcctcaggtaccaagagtctttagaagtcaatcctgtatctcagctacttggtaggctgaggcacaagaatcacttgaacccaggagacagaggttgcagtgagccaagatcaggagactgcactcacagcctgaaggacagagtgagactctcagggccactttaaactcgaagggactcacggactctcacccggacgtctcaatttgctctgggttgagaaagaggggccgcaatttccaggtctgtggggactcaacgtccccggtatagcagcaccacaggactgggaagcacacataaaacag

SEQ ID NO: 15853 - RNA, 5985 nt, Homo sapiens
  source 1..5985: mol_type = other RNA
gctgggattacaggcatgagccagagcacctggtctatttttttttttttaaattaagaaacacgttggtcatggtggctcatggctgtaatcccagcaccttgggaggccaatacggctggatcgcttgagccctggaattcaagaccagctcgggcaacatggtgaaagcccatctctactaggaacacaaaaatttgcccggtgcggtggcacctggctatggtcctagcaactttggaggctgaggtgggaggatcccttgaacccaggagattgaagcttcagtgagggctgatcctgtcaccgctctcatgcctggccaacagaatgagacccatctttaatagaaatgaagaaaaaggaaacacatgcgtcctgggtctggggacagggagagtctaaggccaattaacacgaacctcaggaggtcctgatgacgtgtgtccatggtgttgaggctgcagtttggtttcacacattttacagacacacgagacagcaatcagtacatatatacattggtccggtctggaaaggtggaataactggaattggggaccttctgggtcacaggtagataacaaataacattctttgaatctttgatcagcctttcactaaatacacaatttatatgtgagcagggaggagggataagtcacttatgccttaggctggctcagggaccctgtatttttacataaatagggcaagggaagcaatcagatagacatttgactcaggtgtgcagagggatgggctctttcccacatctgtgaagataagctctcagtttacatcgccagggtgaaattcaacagaactattttagggtggagatcttgaggttcccggtttgggaggggcatatgtagctttttaaaaaatctttgtaactatcttgtttaggaataaaatggaaggcaggtttgtctgacgcagttcccagattgacttttctctttggcttagtaatttttattttcctttcacaagcttgtgacagccataatgctttgacacactgatactgttttatatagatttttccacaacagtaaagtccaagggtctgtcatgaaccgggttagagaagatgagaaaattttcagaagactccatctcaaaaaaacaaaacaaacaaaacagaatttaaaatacagaattaagtcatttgactttttttaaatgaaaagtctcacatatttattactgaaccaagccaacaaaggtgttcataacagatccagagaaaaaaaatacattctcaataaaacatgtccaactctccagatagtggtgacattttcagcttgatatggtaacgtgactgaatcttcagacagcatgaatatgtgtgccatctcatatgcaattccttatagatccagcttggctcttctccagtgtcgtctttgacagttgtacctataaaacttatgtggatggtctgcctgccactctgtgcatcactttcttttttttttttttttttttttttttgagatggagtctcgctctgtcacccaggctggagtgcagtagcatgatctctgctcatggcaagctccacctcctcggttcatgccattctcctgcctcagcctcctgagtagctgggactacaggcgcccacaaccacgcctggctaattttttgtatttttagtagagatggggtttcaccgtgttagccaggattttctcgatctcctgacctcgtgatgctcttgcctcggcctcccaaagtgctgggattacaggtgtgagccaccacacctgtcctgtgcatcactttcaacatcatcttgtcccaacttaaaataagttttccatttacaaactggtgatttattttgggaatcgtccccataaccttttcataaagcatcaatgatttcattgtccctctacccaaactttaccagattcatttttcgatacactatctgtctctgtcacccatgctggagtacaatggcatgatcatggctccctgcagcctcgaactcctaggctcaagccatcctcccactgcagactccacagaagctgaaccagcagacatgtgccacaatgcccagctaatttatgtattttttgtagagaaggtggtttcaccattctgcccaggctggtcttgagtaccggggcccacgtgacccaactgtctcagcctctgaaaattatgggattacaggcctgagccacagcatctggtctcatcgcaaatttgatgtttcttcttgtttcagttttagcagaatttacattgccttgattgagtctcttttcaaactcatgtcttacccatctgagtgcctcaaaccaaaccctgttcagacatgttataacggatttgtatcagtttatcttggtgcaaaaaatgtgatatcatgcacaattttctcataatatgtatttttccatgaacttcctgaagaccccttgtactagcgaactgtattcaagaggttataaaaaggattgttgatatgcaagtgccacttatttctgggatgcaaaatggttcaacatagtcaagcaaatcaatgtgatataccacttgaacataatgaaagatgaaaaccacatcatctcaatacatggagaaaaagcatttcacaaaattcaacatccagtcatcatggaaatcctaaacaaaatagaaagagaaggaaatttacctcaacaatacaaagaccatccatgaaatgaccacagcagaaataaccagtcagggaaaatggaatgcttttcctgtaggatctcacatgatgcaagaatgctctcaccccttctattcaatcaatactggctgtcctagctagagcaatgaaatagcaaaagaaatcaaactcatccaaatcagaaagaaagaagtaaaactatttctttgtagatgacatgatcttctgtgtagaaaatcacaaagagtcaaccaaaatgcaactggaactaaaaaacatatgcagtggatttgaagaatagaataacagcaccaaaaattagttgaatttccatacattaacaataaacaatttaaaaagaaaattaaaaaaacactttcatttgctaaagaacttaaagtaagaaatacttaggaataaatgaaaaaagttgagaagtttctaccttcaaatctacaaacattgatcaaagtgataaaaacatgtgcaaataagagatacaagccatattgaatggaataatattgctaaatgattataactgaatgtgatgtagattcaacacaatacccagagaaatttctataactttttgttaaagaaacaaaaaacaggccaggtgtggtggctcacgcctgtaatctcagcactttggcaggtggaggcaggtggattttaaggacagaagatcgagaccatcctagctaacacggtgaaacccagtctctactaaaaatacaaaaaattacccgggcatggtggcacgcacctgtagtcccagctactcaggagactgaggcaggagaattgcatgaacctgggaggtgaatgttgcagtgaaccgagatcacatcactgcactccaacgtgggcgacagagcaagattccatcttaaaaataaataaataaataaaagaacatacaggctgggaaaagtggctcccgtctgttggccaggctggtctcaaattcatgacctcaagtgacctacctgtcttggcctctcaaagtgctgggattacaggtgtgagacaccacgcctggcccaatcctcttaacataaacagtttaatgtcgattaatgcttgaaatcaatgttaagtcaactcaaactcaggtcaatgctgatttgactctgatgtcaattaatgcttgatggtttgctatactcattgcacttgaaacaattgtctccaaaaggaattttctgatgttctgcaaggagtgacctcagactaaagaccttgccacactgatgacatttgtaagatttctgtccagtatggattctctgatgcctaataaggtgtgaaggtgaattaaaggctttaccacaatcaccacacttgtgaggtttctctcctgtatgaatcctcctatgtctttcaaggtgtgatttgcgaatgtaaactttgtcacattcttcacattcgtaaagtttctctccagtatgaagtttttgatgacatgcgaggtacgcttttgtactaaaaaccttgccacattcattacatgtgtaaggtctctctccagtatgaactctctgatgttctgcaagacgtgaatcactccggaaagccttgtcacaaaccttacatttgtatggtttctctccagtatgaatcctcctatgtctttcaagatgtgatttgcgactgaaaactttgtcgcattcttcacatctgtaaggtttctctccagtgtgaactctacgatgtcctgcaagagttgctcgttgcttaaaaaccttgccacattcattacacttatagggtttctctgcagtatgaactgccttatgaattacgaggactgaatttcgagcgaaggtcttgccacactcattacatttgtaaggtttctctccagtatgcagtctatgatggtacacaaggtgtgatgtctgactaaaggtcttgccacactcattacacttataaggtttctctccagtatgacttctatgatgacatgcaagggttgctttttgatcaaaaaccttgccacattcattacatgtgtaatgtttgtctcccctgtgaattctagtatgttttgccaggtgtgaatcatgcttaaaagccttgtcgcaaaccttacatttgtatggtttctctccagtatgaattatcctatgtatttcaagatgtgatttgcaactgaaaactttctcacattcttcacatttgtaaggtttctctccagtatgaattctcctatgtcttcgcaaatgcaaatgaaatcttgattcaagctgacctttaataggcttgtttccagcatgcctttgatcatatcggtctgtactactagtcaacttttttatttctgtcatgggtgcttcatggtcatttgtttcatcttcttgccactgaaacacaaagtcatgaatgtctttctcaatttcctgggagcaaaatgctccaatgtgataacttgcttgtctctgcaatgtccctgtgtggatcacttctgtattgccttgccctgttgatgacaatgtattcatcatgcatttggaagagatatccagggagaccaggttcctataattctccagcatcacgtctctgtatagagtcctctgagcagggtccaggcatttccactcctcctgagagaattctatggccacatccctgaatgtcagtagaccctgagaaagagccatccccgactcctttgctttcctcttcctcttctgggtttcttcctcaggtaccaagagtctttagaagtcaatcctgtatctcagctacttggtaggctgaggcacaagaatcacttgaacccaggagacagaggttgcagtgagccaagatcaggagactgcactcacagcctgaaggacagagtgagactctcatgcctgtaatcccagcactttgggagggtgaggcggtggatcatgagatcaagaggttgagacaattttggccagcgtggtgaaacccgctctctactacaagtacaaaattagctgggcttctcggcacgcccctgttgtcccagctacttgggagactgaggcaaaagaatcacttgaactcgggagtcagaagttgcagtgagctgagatggcaccagtgcactccagccaggctgaggtgggagaattgcttgagcccggagagcagaggttgaagtgaatcaagatcgcacaactgccctccagcccggacgtctcaatttgctctgggttgagaaagaggggccgcaatttccaggtctgtggggactcaacgtccccggtatagcagcaccacaggactgggaagcacacataaaacag

SEQ ID NO: 15854 - RNA, 5602 nt, Homo sapiens
  source 1..5602: mol_type = other RNA
gctgggattacaggcatgagccagagcacctggtctatttttttttttttaaattaagaaacacgttggtcatggtggctcatggctgtaatcccagcaccttgggaggccaatacggctggatcgcttgagccctggaattcaagaccagctcgggcaacatggtgaaagcccatctctactaggaacacaaaaatttgcccggtgcggtggcacctggctatggtcctagcaactttggaggctgaggtgggaggatcccttgaacccaggagattgaagcttcagtgagggctgatcctgtcaccgctctcatgcctggccaacagaatgagacccatctttaatagaaatgaagaaaaaggaaacacatgcgtcctgggtctggggacagggagagtctaaggccaattaacacgaacctcaggaggtcctgatgacgtgtgtccatggtgttgaggctgcagtttggtttcacacattttacagacacacgagacagcaatcagtacatatatacattggtccggtctggaaaggtggaataactggaattggggaccttctgggtcacaggtagataacaaataacattctttgaatctttgatcagcctttcactaaatacacaatttatatgtgagcagggaggagggataagtcacttatgccttaggctggctcagggaccctgtatttttacataaatagggcaagggaagcaatcagatagacatttgactcaggtgtgcagagggatgggctctttcccacatctgtgaagataagctctcagtttacatcgccagggtgaaattcaacagaactattttagggtggagatcttgaggttcccggtttgggaggggcatatgtagctttttaaaaaatctttgtaactatcttgtttaggaataaaatggaaggcaggtttgtctgacgcagttcccagattgacttttctctttggcttagtaatttttattttcctttcacaagcttgtgacagccataatgctttgacacactgatactgttttatatagatttttccacaacagtaaagtccaagggtctgtcatgaaccgggttagagaagatgagaaaattttcagaagactccatctcaaaaaaacaaaacaaacaaaacagaatttaaaatacagaattaagtcatttgactttttttaaatgaaaagtctcacatatttattactgaaccaagccaacaaaggtgttcataacagatccagagaaaaaaaatacattctcaataaaacatgtccaactctccagatagtggtgacattttcagcttgatatggtaacgtgactgaatcttcagacagcatgaatatgtgtgccatctcatatgcaattccttatagatccagcttggctcttctccagtgtcgtctttgacagttgtacctataaaacttatgtggatggtctgcctgccactctgtgcatcactttcttttttttttttttttttttttttttgagatggagtctcgctctgtcacccaggctggagtgcagtagcatgatctctgctcatggcaagctccacctcctcggttcatgccattctcctgcctcagcctcctgagtagctgggactacaggcgcccacaaccacgcctggctaattttttgtatttttagtagagatggggtttcaccgtgttagccaggattttctcgatctcctgacctcgtgatgctcttgcctcggcctcccaaagtgctgggattacaggtgtgagccaccacacctgtcctgtgcatcactttcaacatcatcttgtcccaacttaaaataagttttccatttacaaactggtgatttattttgggaatcgtccccataaccttttcataaagcatcaatgatttcattgtccctctacccaaactttaccagattcatttttcgatacactatctgtctctgtcacccatgctggagtacaatggcatgatcatggctccctgcagcctcgaactcctaggctcaagccatcctcccactgcagactccacagaagctgaaccagcagacatgtgccacaatgcccagctaatttatgtattttttgtagagaaggtggtttcaccattctgcccaggctggtcttgagtaccggggcccacgtgacccaactgtctcagcctctgaaaattatgggattacaggcctgagccacagcatctggtctcatcgcaaatttgatgtttcttcttgtttcagttttagcagaatttacattgccttgattgagtctcttttcaaactcatgtcttacccatctgagtgcctcaaaccaaaccctgttcagacatgttataacggatttgtatcagtttatcttggtgcaaaaaatgtgatatcatgcacaattttctcataatatgtatttttccatgaacttcctgaagaccccttgtactagcgaactgtattcaagaggttataaaaaggattgttgatatgcaagtgccacttatttctgggatgcaaaatggttcaacatagtcaagcaaatcaatgtgatataccacttgaacataatgaaagatgaaaaccacatcatctcaatacatggagaaaaagcatttcacaaaattcaacatccagtcatcatggaaatcctaaacaaaatagaaagagaaggaaatttacctcaacaatacaaagaccatccatgaaatgaccacagcagaaataaccagtcagggaaaatggaatgcttttcctgtaggatctcacatgatgcaagaatgctctcaccccttctattcaatcaatactggctgtcctagctagagcaatgaaatagcaaaagaaatcaaactcatccaaatcagaaagaaagaagtaaaactatttctttgtagatgacatgatcttctgtgtagaaaatcacaaagagtcaaccaaaatgcaactggaactaaaaaacatatgcagtggatttgaagaatagaataacagcaccaaaaattagttgaatttccatacattaacaataaacaatttaaaaagaaaattaaaaaaacactttcatttgctaaagaacttaaagtaagaaatacttaggaataaatgaaaaaagttgagaagtttctaccttcaaatctacaaacattgatcaaagtgataaaaacatgtgcaaataagagatacaagccatattgaatggaataatattgctaaatgattataactgaatgtgatgtagattcaacacaatacccagagaaatttctataactttttgttaaagaaacaaaaaacaggccaggtgtggtggctcacgcctgtaatctcagcactttggcaggtggaggcaggtggattttaaggacagaagatcgagaccatcctagctaacacggtgaaacccagtctctactaaaaatacaaaaaattacccgggcatggtggcacgcacctgtagtcccagctactcaggagactgaggcaggagaattgcatgaacctgggaggtgaatgttgcagtgaaccgagatcacatcactgcactccaacgtgggcgacagagcaagattccatcttaaaaataaataaataaataaaagaacatacaggctgggaaaagtggctcccgtctgttggccaggctggtctcaaattcatgacctcaagtgacctacctgtcttggcctctcaaagtgctgggattacaggtgtgagacaccacgcctggcccaatcctcttaacataaacagtttaatgtcgattaatgcttgaaatcaatgttaagtcaactcaaactcaggtcaatgctgatttgactctgatgtcaattaatgcttgatggtttgctatactcattgcacttgaaacaattgtctccaaaaggaattttctgatgttctgcaaggagtgacctcagactaaagaccttgccacactgatgacatttgtaagatttctgtccagtatggattctctgatgcctaataaggtgtgaaggtgaattaaaggctttaccacaatcaccacacttgtgaggtttctctcctgtatgaatcctcctatgtctttcaaggtgtgatttgcgaatgtaaactttgtcacattcttcacattcgtaaagtttctctccagtatgaagtttttgatgacatgcgaggtacgcttttgtactaaaaaccttgccacattcattacatgtgtaaggtctctctccagtatgaactctctgatgttctgcaagacgtgaatcactccggaaagccttgtcacaaaccttacatttgtatggtttctctccagtatgaatcctcctatgtctttcaagatgtgatttgcgactgaaaactttgtcgcattcttcacatctgtaaggtttctctccagtgtgaactctacgatgtcctgcaagagttgctcgttgcttaaaaaccttgccacattcattacacttatagggtttctctgcagtatgaactgccttatgaattacgaggactgaatttcgagcgaaggtcttgccacactcattacatttgtaaggtttctctccagtatgcagtctatgatggtacacaaggtgtgatgtctgactaaaggtcttgccacactcattacacttataaggtttctctccagtatgacttctatgatgacatgcaagggttgctttttgatcaaaaaccttgccacattcattacatgtgtaatgtttgtctcccctgtgaattctagtatgttttgccaggtgtgaatcatgcttaaaagccttgtcgcaaaccttacatttgtatggtttctctccagtatgaattatcctatgtatttcaagatgtgatttgcaactgaaaactttctcacattcttcacatttgtaaggtttctctccagtatgaattctcctatgtcttcgcaaatgcaaatgaaatcttgattcaagctgacctttaataggcttgtttccagcatgcctttgatcatatcggtctgtactactagtcaacttttttatttctgtcatgggtgcttcatggtcatttgtttcatcttcttgccactgaaacacaaagtcatgaatgtctttctcaatttcctgggagcaaaatgctccaatgtgataacttgcttgtctctgcaatgtccctgtgtggatcacttctgtattgccttgccctgttgatgacaatgtattcatcatgcatttggaagagatatccagggagaccaggttcctataattctccagcatcacgtctctgtatagagtcctctgagcagggtccaggcatttccactcctcctgagagaattctatggccacatccctgaatgtcagtagaccctgagaaagagccatccccgactcctttgctttcctcttcctcttctgggtttcttcctcaggtaccaagagtctttagaagtcaatcctgtatctcagctacttggtaggctgaggcacaagaatcacttgaacccaggagacagaggttgcagtgagccaagatcaggagactgcactcacagcctgaaggacagagtgagactgcgctgtggtgtgaccttcagtccctgccatccgcttccgggtctat

SEQ ID NO: 15855 - RNA, 5484 nt, Homo sapiens
  source 1..5484: mol_type = other RNA
gctgggattacaggcatgagccagagcacctggtctatttttttttttttaaattaagaaacacgttggtcatggtggctcatggctgtaatcccagcaccttgggaggccaatacggctggatcgcttgagccctggaattcaagaccagctcgggcaacatggtgaaagcccatctctactaggaacacaaaaatttgcccggtgcggtggcacctggctatggtcctagcaactttggaggctgaggtgggaggatcccttgaacccaggagattgaagcttcagtgagggctgatcctgtcaccgctctcatgcctggccaacagaatgagacccatctttaatagaaatgaagaaaaaggaaacacatgcgtcctgggtctggggacagggagagtctaaggccaattaacacgaacctcaggaggtcctgatgacgtgtgtccatggtgttgaggctgcagtttggtttcacacattttacagacacacgagacagcaatcagtacatatatacattggtccggtctggaaaggtggaataactggaattggggaccttctgggtcacaggtagataacaaataacattctttgaatctttgatcagcctttcactaaatacacaatttatatgtgagcagggaggagggataagtcacttatgccttaggctggctcagggaccctgtatttttacataaatagggcaagggaagcaatcagatagacatttgactcaggtgtgcagagggatgggctctttcccacatctgtgaagataagctctcagtttacatcgccagggtgaaattcaacagaactattttagggtggagatcttgaggttcccggtttgggaggggcatatgtagctttttaaaaaatctttgtaactatcttgtttaggaataaaatggaaggcaggtttgtctgacgcagttcccagattgacttttctctttggcttagtaatttttattttcctttcacaagcttgtgacagccataatgctttgacacactgatactgttttatatagatttttccacaacagtaaagtccaagggtctgtcatgaaccgggttagagaagatgagaaaattttcagaagactccatctcaaaaaaacaaaacaaacaaaacagaatttaaaatacagaattaagtcatttgactttttttaaatgaaaagtctcacatatttattactgaaccaagccaacaaaggtgttcataacagatccagagaaaaaaaatacattctcaataaaacatgtccaactctccagatagtggtgacattttcagcttgatatggtaacgtgactgaatcttcagacagcatgaatatgtgtgccatctcatatgcaattccttatagatccagcttggctcttctccagtgtcgtctttgacagttgtacctataaaacttatgtggatggtctgcctgccactctgtgcatcactttcttttttttttttttttttttttttttgagatggagtctcgctctgtcacccaggctggagtgcagtagcatgatctctgctcatggcaagctccacctcctcggttcatgccattctcctgcctcagcctcctgagtagctgggactacaggcgcccacaaccacgcctggctaattttttgtatttttagtagagatggggtttcaccgtgttagccaggattttctcgatctcctgacctcgtgatgctcttgcctcggcctcccaaagtgctgggattacaggtgtgagccaccacacctgtcctgtgcatcactttcaacatcatcttgtcccaacttaaaataagttttccatttacaaactggtgatttattttgggaatcgtccccataaccttttcataaagcatcaatgatttcattgtccctctacccaaactttaccagattcatttttcgatacactatctgtctctgtcacccatgctggagtacaatggcatgatcatggctccctgcagcctcgaactcctaggctcaagccatcctcccactgcagactccacagaagctgaaccagcagacatgtgccacaatgcccagctaatttatgtattttttgtagagaaggtggtttcaccattctgcccaggctggtcttgagtaccggggcccacgtgacccaactgtctcagcctctgaaaattatgggattacaggcctgagccacagcatctggtctcatcgcaaatttgatgtttcttcttgtttcagttttagcagaatttacattgccttgattgagtctcttttcaaactcatgtcttacccatctgagtgcctcaaaccaaaccctgttcagacatgttataacggatttgtatcagtttatcttggtgcaaaaaatgtgatatcatgcacaattttctcataatatgtatttttccatgaacttcctgaagaccccttgtactagcgaactgtattcaagaggttataaaaaggattgttgatatgcaagtgccacttatttctgggatgcaaaatggttcaacatagtcaagcaaatcaatgtgatataccacttgaacataatgaaagatgaaaaccacatcatctcaatacatggagaaaaagcatttcacaaaattcaacatccagtcatcatggaaatcctaaacaaaatagaaagagaaggaaatttacctcaacaatacaaagaccatccatgaaatgaccacagcagaaataaccagtcagggaaaatggaatgcttttcctgtaggatctcacatgatgcaagaatgctctcaccccttctattcaatcaatactggctgtcctagctagagcaatgaaatagcaaaagaaatcaaactcatccaaatcagaaagaaagaagtaaaactatttctttgtagatgacatgatcttctgtgtagaaaatcacaaagagtcaaccaaaatgcaactggaactaaaaaacatatgcagtggatttgaagaatagaataacagcaccaaaaattagttgaatttccatacattaacaataaacaatttaaaaagaaaattaaaaaaacactttcatttgctaaagaacttaaagtaagaaatacttaggaataaatgaaaaaagttgagaagtttctaccttcaaatctacaaacattgatcaaagtgataaaaacatgtgcaaataagagatacaagccatattgaatggaataatattgctaaatgattataactgaatgtgatgtagattcaacacaatacccagagaaatttctataactttttgttaaagaaacaaaaaacaggccaggtgtggtggctcacgcctgtaatctcagcactttggcaggtggaggcaggtggattttaaggacagaagatcgagaccatcctagctaacacggtgaaacccagtctctactaaaaatacaaaaaattacccgggcatggtggcacgcacctgtagtcccagctactcaggagactgaggcaggagaattgcatgaacctgggaggtgaatgttgcagtgaaccgagatcacatcactgcactccaacgtgggcgacagagcaagattccatcttaaaaataaataaataaataaaagaacatacaggctgggaaaagtggctcccgtctgttggccaggctggtctcaaattcatgacctcaagtgacctacctgtcttggcctctcaaagtgctgggattacaggtgtgagacaccacgcctggcccaatcctcttaacataaacagtttaatgtcgattaatgcttgaaatcaatgttaagtcaactcaaactcaggtcaatgctgatttgactctgatgtcaattaatgcttgatggtttgctatactcattgcacttgaaacaattgtctccaaaaggaattttctgatgttctgcaaggagtgacctcagactaaagaccttgccacactgatgacatttgtaagatttctgtccagtatggattctctgatgcctaataaggtgtgaaggtgaattaaaggctttaccacaatcaccacacttgtgaggtttctctcctgtatgaatcctcctatgtctttcaaggtgtgatttgcgaatgtaaactttgtcacattcttcacattcgtaaagtttctctccagtatgaagtttttgatgacatgcgaggtacgcttttgtactaaaaaccttgccacattcattacatgtgtaaggtctctctccagtatgaactctctgatgttctgcaagacgtgaatcactccggaaagccttgtcacaaaccttacatttgtatggtttctctccagtatgaatcctcctatgtctttcaagatgtgatttgcgactgaaaactttgtcgcattcttcacatctgtaaggtttctctccagtgtgaactctacgatgtcctgcaagagttgctcgttgcttaaaaaccttgccacattcattacacttatagggtttctctgcagtatgaactgccttatgaattacgaggactgaatttcgagcgaaggtcttgccacactcattacatttgtaaggtttctctccagtatgcagtctatgatggtacacaaggtgtgatgtctgactaaaggtcttgccacactcattacacttataaggtttctctccagtatgacttctatgatgacatgcaagggttgctttttgatcaaaaaccttgccacattcattacatgtgtaatgtttgtctcccctgtgaattctagtatgttttgccaggtgtgaatcatgcttaaaagccttgtcgcaaaccttacatttgtatggtttctctccagtatgaattatcctatgtatttcaagatgtgatttgcaactgaaaactttctcacattcttcacatttgtaaggtttctctccagtatgaattctcctatgtcttcgcaaatgcaaatgaaatcttgattcaagctgacctttaataggcttgtttccagcatgcctttgatcatatcggtctgtactactagtcaacttttttatttctgtcatgggtgcttcatggtcatttgtttcatcttcttgccactgaaacacaaagtcatgaatgtctttctcaatttcctgggagcaaaatgctccaatgtgataacttgcttgtctctgcaatgtccctgtgtggatcacttctgtattgccttgccctgttgatgacaatgtattcatcatgcatttggaagagatatccagggagaccaggttcctataattctccagcatcacgtctctgtatagagtcctctgagcagggtccaggcatttccactcctcctgagagaattctatggccacatccctgaatgtcagtagaccctgagaaagagccatccccgactcctttgctttcctcttcctcttctgggtttcttcctcaggtaccaagagtctttagaagtcaatcgcgctgtggtgtgaccttcagtccctgccatccgcttccgggtctat

SEQ ID NO: 15856 - RNA, 7566 nt, Homo sapiens
  source 1..7566: mol_type = other RNA
gctgggattacaggcatgagccagcacacctggcaatttgtctgctgtttagtggaggacagcagcaagaaatgtatcctcataatcaaacaactggaataagaagtagaaactacactacagccctattttgtgaccaaaattacgttttagctgatagcatagaaaatgtgctggcaaaatgtgtaatgttacggatattgcttggtgattcctttttctcaattcagggcctatcagctaacttttaccttgcgtaccttctggtaatcaggtgaggactaggaatggtcaagtgcagtagtaacttgctgtccctggaagcactctttccagaagcctaataatttgaaatagtgcccaaagaactggggaagagttacaagcctgggagaaaaaaacctactaagaaaaaaaaacttagctaaagaaatgaatgcctctggccgtgcgcggtggctcgtgcctgtaatcctagctctttgggaggctgtggcgggcagatcacgaggtcaagagttcgagaccaacctggccagcatggtgaaacttcgtctctactaaaaatacaaaaattagccaagcatggtggtgtgcgcctgtagtcccagtactcgggaggctgaggcaggagactcgcttgaacacgggaggtggaggttgcagtaagccgagattgtgccagtgcactccagcctgggcaacagagtgagactccgtctcaaaaaaaacaaaacaaaaaacacctctctctttcactctctctcatgcacgtgcacacacacacacacacacacacacaccacacaaactgcatggtacatgttatccaaaggctgaatttctttggactgaatatcactagaagtttatataattgctctatattagctaaaactaataatcatgtaccaaaaatatacttttttttttttttacaaaataacacaatttattaccattttgaaacaaatcacaaaataacattcagaaactcaacatttctaaataacttaattcacaataagtttagtcataaagtcatgctacaaaactcctgtgtataaaagattattaccaaggtattcatagatgttaaaatgttcttcagaatggagttggttctagaagccaaagattctggaatgatgctcgtaatcatgactgccagcctgggagaggagctggctatgcgcatgtgctcttagcttccaactcaccagtcttttgatgggagtgatccctccaggcagtagcacctcagaggcaggtaccctactgatcacagaggcaaagagcctcccacccatataatgttagacaactctacattcatttaaaatctagaggtgggaatgataattcgcaaagcttctattctgagtaggagaactacttgacacatcccccagagggatgatcttggatgtaacagacatggaagacgactcaagtagggaaaaagggaaatcctgactctgattatgtcaaaagacagttaactactcatgtgggtttagaacgagcaagggtgaggtttgattctctaacatccaagtgcaggctagatatttacccatctgccctatggaagtcctttccaccaacatccagttcctaagtttaaagtgcaaatctactgaaaaatagtttactatccctcttcccctatgttaaatttgctagatcataatttggttggctgggtctcctctaaactgcccaatatgggaaattaactagaatccagttaatgacttctccaaatatcaagtaaaaagttttatcagtttatcttaggtcagagaaaggtaagactcagtctagttcttcctttcagttttcttcctttacagatttataaaatgcaggaatagagatacagatatggtatttctaaaagttccatgattttaaaacatgacccttgatttttggaagttcacccattttatggtttacaaaaagaaaacaatatgacacatgttagagcacagataaagaaatatggtcaagttagcttgtcagaagaagcaccaactctgctacactgaatcttgcttttatatttcatgatttacagacacattaaacagccccaaataaataaaatctgtgccaaaggaatgaatttctagtaaagggtaacatgcaatttagcagttttcttcctttaccaacacttacagagtataaggtcttagtgaattgatggtctgactgtagtcagagagacataatctattcatgactgatgctttgacacttcctcctaatgcttttaagtgaatgattaactccaacctttctgggccctgtgcttttccatttagccctgagaaaaacccaggtagaagattccaactctctttacacatcaccaattctcagaataagtcaacagtcaagattcatttcttattcttccttattctgcttcagaccactggtaaaaggtgtcaaaagaagtgtttattcaagttcaaattcctctttccacaaaagaaccacatttttttttttctttttgagacggagacttactctgtcacccaggctggagtacagtcacactatttcggctcactgaagcctctgcctcccgggttcaagcaattctcctgcctcagcctcccgagtagctgggattacaggcatgcgccaccacgcccggctatctttttatatttttggtagacatggggtttcaccacgttggccaggctggcctcgaactcctgacctcaagtgatctgcccaccacggcctcccaaagtgctgggattacaggcatgagccacagtgcccaatcaggaaacacatttaagtgccttatactaccatatgtggaatgaatccagtagccataccaagttattgaccagttatcttaagcagacattcttctgatcacatccaaaattgatgtctacatcagctaactttcctacaagattatcaaattttacacagtatttttctgtatttaatgactgccatggtctgcaaaattatgtgattagacaatgaatgacgcttaaagaatgatgacctattttctaaagtacactcaaaatattaaactttagagacaaagcaaaatctatcataaagttggcttctgttgatagaaacagagaggtaggttaataatcactgtcctaagataagcaagaatgcttagaaataaaagttgagaccctgcttcaaaaaagagaagttgaaccttccagccctgagtttctaatattacatgaaaattatgaaaatgagcattaagccagtcgcagtggctcacgtctgtaatcccagcactttgggaggctgaggcaggcggatcacgaggtcaggagtttgagaccagcctggccaatatggtgaaacgccgtctgtactaaaaatacaaaaattagccaggcatggtggcgcgtgcctgtagtcccagctacttgggaggcggaggcagaagaattgcttgaacccgggagacggaggttgcagtgagctgagattgcgccactgcactccagcctaggtaacagagcgagactctgtctcaaaaaaaaaaaaaaatgagcattacaaaaaataccagtgaccatttctttccatccatgattactgaatacatcaccttctctcatataacaattcaagtggcacatggctacagactgaaaataaatggaccctggacacaagtgatgttggtataaaaagtacaactaagggagaatttgttcccaccctcctacccaagggacagatggcaatgtctggagatatctttgttgtcatggctgaggagggggtctactggaatctagtgggtagaggccagggctgcagctgaacatcctaagcacacaggacagcccccaacaacaatgaattatcaatcccaaaatgttaatagttccaaggttgatcctctggtttaaaggaacaaattcttattaacagagaacaacacaaaaaccttttaaggcctgtctaggtaatacagccctaatcttagagttagggaacatagaaaagttaaactccttggtagactaaaatcaaatttgctgtgaaaaactaaaatactggactgattccagagttttaccatcacttacaagaatagaagaaatttggccaggcacggtggctcatgcctgtaatcccagcactttgggaggccgatgtgggcaggtcatctgaagttaggagttcaagacaagcctggccaacatggtgaaaccccatctctactaaaaatacaaaaataggccaggcatgatggcacgtgcctgtggtcccagctactcgggagtgagactctgtttaaaacaaacaaacaaacaaacaaaaaaaaacagaatagaaaaaatttaaatgatccactaaaatggcgtaatgtcttaaaccggaagcacagagataatctattccacataggtcaaatatctgatccaagaggcataaaccaaaggcagttttatcagctaaatttgcagcagtaaaggataatttagggaatgatttgagagaatatcctacatttcttcatacatcccaactgccattttctaatggcatgggttccatgaacagggatgcatagaagtcattcaaagatttgttgaatgatactgaatatgaattttgcatgaaatggacagagaaaagtatcttacatttgtctgagaactacctgtaattaaaagtcattgagaaacaaggagaaagagaaccagtttctatattacagaattcagaaaaaacaaacaccaaaactctaagccattttacaaataaattcaatatgaaatcacttacttcctattatattcacttccagggttacttttagaaaacatatccatatcaacatggcttcaagcttgcctactgaaggaagtgcaaactttaagaagatcatcttccctctcagtttatggaacttaaaacatcaccaaggagaatgaaggctcattgcctatggttcataaaagaaatgtccaaaggctttgaatgcataaaccagctagagtagaataaggtttcttcctatcagattgaaaagaagagagaaaagaaaactaaaagggtgttagaccaagttttcctcttttttttttttttttttttttaaatatggagtctcgctctattgcccaggctggagtgcaatggcgcaatctcggctcactgcaacctccgcctcccgggttcaaatgattctcctgcctcagcctcccgagtagttgggactacaggcgcccaccaccaggactggctaatttttgtatttttagtagagacggggtttcaccatgttggtcaggctggtcttgaactcctgatctcagatgatccgcccgcctcggcctcccaaagtgctgggatgacaggcatgagccaccacgcctggcctcttgtttgtatttagagttgattgtcaaagcagtggtcccttttgatcagagtaacttagaaaaatcaagtaattcctatgtaaatgatagctgaaatcttctgaaacccaggactacttatgcaatcactttttaaagatgattcttccctctttcactgtgattttatgcaagtaaaatcacacaagtagatggggaaaccagaatcaacagtctctgagggactttaggcacaatttggcagagggcccctgacttcttttctgcaatctaatagtgatccagccatggcctcctatgacctcatctgcttactgactacaatgtcttacattttcctgaaggattttttgtttacatgataaattctaacctctgcatctaactattgctttgcaattttgaggttaaatcacctacactgctttatgtaggagacaatcctcaaacatattgccatttgcctgggatctcataatgaaacatctcccttccctccacaaccacgtacataatacattttaagagctgtttaacttagaacttctcaaaaaatatattttgaaatactaagtttcattatacccttacttataaccatggtagtcacttttcccaacaatgagggtcaccagaccaaataattagggtaaattttgacatacatcaatggccagcatttagtctaggaattcaaatataactaatgctttaaacacataaggaactataaaaccaaaatgtgtgcttaaggcgaggtccacatgagtaacattgccacattatcagtcaaagaaatgatcatgacagtcattttaaccactaactgagatcacagaatgactgtacacaatgactcaagtggccatgcatataaaaacaacctaaattccagttgacaatgtgcacatttttggaaaaacaaataagtataatatagactagaaggtctctgagatactactttttccttttttcaccatatcttttccaatggaactttggagtcttggttccggacctgctgtatttctaagaggaactcttcccatcaccatgctgccttctgagctaaaggcatgtgcttctgaattgtacagagacagaccttcaggaaaaatgttctgaattttcaaatgtacatcttttaaaatgtctaacctaaaaaaaatgaacaaactgaaaaaaacatttgttcctttgttattaaaaatgactggtctacaaaggttttgttttagtagatggggctacacagtacgtaactgagactgaagacaaaaatcgaaaatttgtggtttctaaaaagagaaataggatatataaggttggcattaccagttttggggagaaacactgaataagttaaaggaaaaaaaaagatgagaatgagtgatctgttttatcttaagaaacttttgtcccatacagaatctttaaaatagacaattatataaaatttatctattgttcttatgacatttaaataagttaacacacagtggaaagcgtggcattagttgtcttcttcctcatcccctttaattactggagtaccatccagctttttcagtttgggcactctcttggttgcttcttcaatccagttattctcagcagaatgtttctcttccaagggattgcctacaaacaccaggtcttcgaggcatggcagttctgccagcttcacaaactcagcccagtcttttaccaggttattagacatgtagagaatcttcaatttcttcattatgtggatccctttcaacttctcaataaaattgtaggagatccacagttcttctaatgtgtcccctactgcctccagtccatttaagttctttatgttgtttcttcctaaagataatatcctcaagttttttaagccattcaggttggcaattttttcaatgcagtttgtagacagtgaaagcttctcgcaattagcaagcatggacaaggatgcatccatcttctctatagggggaatctgggcataaagttttatctctttggcttcagatggcctctggccagttttctcttcccatctcgctaaggcttctttgattgttgttgctttcgccattccggcggttgctactgtcactgctctggttgctagggcccgcggggtcagtgc

SEQ ID NO: 15857 - RNA, 7612 nt, Homo sapiens
  source 1..7612: mol_type = other RNA
gctgggattacaggcatgagccagcacacctggcaatttgtctgctgtttagtggaggacagcagcaagaaatgtatcctcataatcaaacaactggaataagaagtagaaactacactacagccctattttgtgaccaaaattacgttttagctgatagcatagaaaatgtgctggcaaaatgtgtaatgttacggatattgcttggtgattcctttttctcaattcagggcctatcagctaacttttaccttgcgtaccttctggtaatcaggtgaggactaggaatggtcaagtgcagtagtaacttgctgtccctggaagcactctttccagaagcctaataatttgaaatagtgcccaaagaactggggaagagttacaagcctgggagaaaaaaacctactaagaaaaaaaaacttagctaaagaaatgaatgcctctggccgtgcgcggtggctcgtgcctgtaatcctagctctttgggaggctgtggcgggcagatcacgaggtcaagagttcgagaccaacctggccagcatggtgaaacttcgtctctactaaaaatacaaaaattagccaagcatggtggtgtgcgcctgtagtcccagtactcgggaggctgaggcaggagactcgcttgaacacgggaggtggaggttgcagtaagccgagattgtgccagtgcactccagcctgggcaacagagtgagactccgtctcaaaaaaaacaaaacaaaaaacacctctctctttcactctctctcatgcacgtgcacacacacacacacacacacacacaccacacaaactgcatggtacatgttatccaaaggctgaatttctttggactgaatatcactagaagtttatataattgctctatattagctaaaactaataatcatgtaccaaaaatatacttttttttttttttacaaaataacacaatttattaccattttgaaacaaatcacaaaataacattcagaaactcaacatttctaaataacttaattcacaataagtttagtcataaagtcatgctacaaaactcctgtgtataaaagattattaccaaggtattcatagatgttaaaatgttcttcagaatggagttggttctagaagccaaagattctggaatgatgctcgtaatcatgactgccagcctgggagaggagctggctatgcgcatgtgctcttagcttccaactcaccagtcttttgatgggagtgatccctccaggcagtagcacctcagaggcaggtaccctactgatcacagaggcaaagagcctcccacccatataatgttagacaactctacattcatttaaaatctagaggtgggaatgataattcgcaaagcttctattctgagtaggagaactacttgacacatcccccagagggatgatcttggatgtaacagacatggaagacgactcaagtagggaaaaagggaaatcctgactctgattatgtcaaaagacagttaactactcatgtgggtttagaacgagcaagggtgaggtttgattctctaacatccaagtgcaggctagatatttacccatctgccctatggaagtcctttccaccaacatccagttcctaagtttaaagtgcaaatctactgaaaaatagtttactatccctcttcccctatgttaaatttgctagatcataatttggttggctgggtctcctctaaactgcccaatatgggaaattaactagaatccagttaatgacttctccaaatatcaagtaaaaagttttatcagtttatcttaggtcagagaaaggtaagactcagtctagttcttcctttcagttttcttcctttacagatttataaaatgcaggaatagagatacagatatggtatttctaaaagttccatgattttaaaacatgacccttgatttttggaagttcacccattttatggtttacaaaaagaaaacaatatgacacatgttagagcacagataaagaaatatggtcaagttagcttgtcagaagaagcaccaactctgctacactgaatcttgcttttatatttcatgatttacagacacattaaacagccccaaataaataaaatctgtgccaaaggaatgaatttctagtaaagggtaacatgcaatttagcagttttcttcctttaccaacacttacagagtataaggtcttagtgaattgatggtctgactgtagtcagagagacataatctattcatgactgatgctttgacacttcctcctaatgcttttaagtgaatgattaactccaacctttctgggccctgtgcttttccatttagccctgagaaaaacccaggtagaagattccaactctctttacacatcaccaattctcagaataagtcaacagtcaagattcatttcttattcttccttattctgcttcagaccactggtaaaaggtgtcaaaagaagtgtttattcaagttcaaattcctctttccacaaaagaaccacatttttttttttctttttgagacggagacttactctgtcacccaggctggagtacagtcacactatttcggctcactgaagcctctgcctcccgggttcaagcaattctcctgcctcagcctcccgagtagctgggattacaggcatgcgccaccacgcccggctatctttttatatttttggtagacatggggtttcaccacgttggccaggctggcctcgaactcctgacctcaagtgatctgcccaccacggcctcccaaagtgctgggattacaggcatgagccacagtgcccaatcaggaaacacatttaagtgccttatactaccatatgtggaatgaatccagtagccataccaagttattgaccagttatcttaagcagacattcttctgatcacatccaaaattgatgtctacatcagctaactttcctacaagattatcaaattttacacagtatttttctgtatttaatgactgccatggtctgcaaaattatgtgattagacaatgaatgacgcttaaagaatgatgacctattttctaaagtacactcaaaatattaaactttagagacaaagcaaaatctatcataaagttggcttctgttgatagaaacagagaggtaggttaataatcactgtcctaagataagcaagaatgcttagaaataaaagttgagaccctgcttcaaaaaagagaagttgaaccttccagccctgagtttctaatattacatgaaaattatgaaaatgagcattaagccagtcgcagtggctcacgtctgtaatcccagcactttgggaggctgaggcaggcggatcacgaggtcaggagtttgagaccagcctggccaatatggtgaaacgccgtctgtactaaaaatacaaaaattagccaggcatggtggcgcgtgcctgtagtcccagctacttgggaggcggaggcagaagaattgcttgaacccgggagacggaggttgcagtgagctgagattgcgccactgcactccagcctaggtaacagagcgagactctgtctcaaaaaaaaaaaaaaatgagcattacaaaaaataccagtgaccatttctttccatccatgattactgaatacatcaccttctctcatataacaattcaagtggcacatggctacagactgaaaataaatggaccctggacacaagtgatgttggtataaaaagtacaactaagggagaatttgttcccaccctcctacccaagggacagatggcaatgtctggagatatctttgttgtcatggctgaggagggggtctactggaatctagtgggtagaggccagggctgcagctgaacatcctaagcacacaggacagcccccaacaacaatgaattatcaatcccaaaatgttaatagttccaaggttgatcctctggtttaaaggaacaaattcttattaacagagaacaacacaaaaaccttttaaggcctgtctaggtaatacagccctaatcttagagttagggaacatagaaaagttaaactccttggtagactaaaatcaaatttgctgtgaaaaactaaaatactggactgattccagagttttaccatcacttacaagaatagaagaaatttggccaggcacggtggctcatgcctgtaatcccagcactttgggaggccgatgtgggcaggtcatctgaagttaggagttcaagacaagcctggccaacatggtgaaaccccatctctactaaaaatacaaaaataggccaggcatgatggcacgtgcctgtggtcccagctactcgggagtgagactctgtttaaaacaaacaaacaaacaaacaaaaaaaaacagaatagaaaaaatttaaatgatccactaaaatggcgtaatgtcttaaaccggaagcacagagataatctattccacataggtcaaatatctgatccaagaggcataaaccaaaggcagttttatcagctaaatttgcagcagtaaaggataatttagggaatgatttgagagaatatcctacatttcttcatacatcccaactgccattttctaatggcatgggttccatgaacagggatgcatagaagtcattcaaagatttgttgaatgatactgaatatgaattttgcatgaaatggacagagaaaagtatcttacatttgtctgagaactacctgtaattaaaagtcattgagaaacaaggagaaagagaaccagtttctatattacagaattcagaaaaaacaaacaccaaaactctaagccattttacaaataaattcaatatgaaatcacttacttcctattatattcacttccagggttacttttagaaaacatatccatatcaacatggcttcaagcttgcctactgaaggaagtgcaaactttaagaagatcatcttccctctcagtttatggaacttaaaacatcaccaaggagaatgaaggctcattgcctatggttcataaaagaaatgtccaaaggctttgaatgcataaaccagctagagtagaataaggtttcttcctatcagattgaaaagaagagagaaaagaaaactaaaagggtgttagaccaagttttcctcttttttttttttttttttttttaaatatggagtctcgctctattgcccaggctggagtgcaatggcgcaatctcggctcactgcaacctccgcctcccgggttcaaatgattctcctgcctcagcctcccgagtagttgggactacaggcgcccaccaccaggactggctaatttttgtatttttagtagagacggggtttcaccatgttggtcaggctggtcttgaactcctgatctcagatgatccgcccgcctcggcctcccaaagtgctgggatgacaggcatgagccaccacgcctggcctcttgtttgtatttagagttgattgtcaaagcagtggtcccttttgatcagagtaacttagaaaaatcaagtaattcctatgtaaatgatagctgaaatcttctgaaacccaggactacttatgcaatcactttttaaagatgattcttccctctttcactgtgattttatgcaagtaaaatcacacaagtagatggggaaaccagaatcaacagtctctgagggactttaggcacaatttggcagagggcccctgacttcttttctgcaatctaatagtgatccagccatggcctcctatgacctcatctgcttactgactacaatgtcttacattttcctgaaggattttttgtttacatgataaattctaacctctgcatctaactattgctttgcaattttgaggttaaatcacctacactgctttatgtaggagacaatcctcaaacatattgccatttgcctgggatctcataatgaaacatctcccttccctccacaaccacgtacataatacattttaagagctgtttaacttagaacttctcaaaaaatatattttgaaatactaagtttcattatacccttacttataaccatggtagtcacttttcccaacaatgagggtcaccagaccaaataattagggtaaattttgacatacatcaatggccagcatttagtctaggaattcaaatataactaatgctttaaacacataaggaactataaaaccaaaatgtgtgcttaaggcgaggtccacatgagtaacattgccacattatcagtcaaagaaatgatcatgacagtcattttaaccactaactgagatcacagaatgactgtacacaatgactcaagtggccatgcatataaaaacaacctaaattccagttgacaatgtgcacatttttggaaaaacaaataagtataatatagactagaaggtctctgagatactactttttccttttttcaccatatcttttccaatggaactttggagtcttggttccggacctgctgtatttctaagaggaactcttcccatcaccatgctgccttctgagctaaaggcatgtgcttctgaattgtacagagacagaccttcaggaaaaatgttctgaattttcaaatgtacatcttttaaaatgtctaacctaaaaaaaatgaacaaactgaaaaaaacatttgttcctttgttattaaaaatgactggtctacaaaggttttgttttagtagatggggctacacagtacgtaactgagactgaagacaaaaatcgaaaatttgtggtttctaaaaagagaaataggatatataaggttggcattaccagttttggggagaaacactgaataagttaaaggaaaaaaaaagatgagaatgagtgatctgttttatcttaagaaacttttgtcccatacagaatctttaaaatagacaattatataaaatttatctattgttcttatgacatttaaataagttaacacacagtggaaagcgtggcattagttgtcttcttcctcatcccctttaattactggagtaccatccagctttttcagtttgggcactctcttggttgcttcttcaatccagttattctcagcagaatgtttctcttccaagggattgcctacaaacaccaggtcttcgaggcatggcagttctgccagcttcacaaactcagcccagtcttttaccaggttattagacatgtagagaatcttcaatttcttcattatgtggatccctttcaacttctcaataaaattgtaggagatccacagttcttctaatgtgtcccctactgcctccagtccatttaagttctttatgttgtttcttcctaaagataatatcctcaagttttttaagccattcaggttggcaattttttcaatgcagtttgtagacagtgaaagcttctcgcaattagcaagcatggacaaggatgcatccatcttctctatagggggaatctgggcataaagttttatctctttggcttcagatggcctctggccagttttctcttcccatctcgctaaggcttctttgattgttgttgctttcgcctgaatcaaccaatcagctcacttgactcaaccaatcaaggcccagcattccggcggttgctactgtcactgctctggttgctagggcccgcggggtcagtgc

SEQ ID NO: 15858 - RNA, 8605 nt, Homo sapiens
  source 1..8605: mol_type = other RNA
gctgggattacaggcatgagccagcagtcctggcaaggagataattttatttatttatttatttagttagttagttagttacttattttttgagatggagtcttgctctgtcacccaggctggagtgcaatggtgccatctccgctcactgcaacctctgcctcccgggctcaagtgatttgcctgcctcagcctcctgagtagctgggattacaggtgtgcaccaacatgcccagatttttattgtatttttagtagaaatggggtttcaccatgttggctaagctggtatcaaactcctgacttcaggtgatctgcctgcctcagtctcccaaagtgctaggattagaggtatgagccaccacgcctggccaaggagataattttaaatgatcaaaatttttggaggcatatcatacatgtacatgtatgatctctgaaaactgttttaaagataaagtcagcaaagtacagcctgttggccaaatctgacccaccacctgttcttgtaatgctgtgaactgagaatagcttttgcatttttaaattttaaaaggttgaaaaaaatcaaaagaagaataaaattttataatatgtgaaaattacctgaatttcaaatgtcagtgtccataaataaggttttattgaagcacagctcacccatccgttatgtaccagctgcattcatgctataatagcagagctgagtggttatgacagagactttctggccaagaaagcctaatgtacttactagctggctctttccagagactgtttgtcaaccctgttttaagagctttcctctaaagaagcacaagcctttagtaaactgaagacttcttcataaagattttctgtgtcagtgatacattatgttaaaaaaagaaaatccatgaatttagtaaagataacattgatattatagactaaaacaataggcatgactttaattatatttaggatgcttattttcccaccttatttcagtagcatagttataagaacacacgctttagggtgatcattcttttttcttgaattttgttgagctttgcatgaccttggactagttacctaacctcttgtaagcctcaggtttcctacaagaacagaataatagcaataccaacctcatgggagtatggtaagtaccaaaatggataagtggggcatttttgggggggaattacttagcttgttatctggtagtaggtgtgcaatagattataattatcatcattctctgaaaatgtcatttttgctttctggtgctccatttctagtactgcctgtaaggtctattttgacaaggaaatctgtaagaccctgccaacatcattttgcatagcaagagcccttctctgtgttacaatctggacaaaaactgtcctcagttgcatgaatccaagaatacacttgacagaagaatggaaaaaaggaagcctaggaagtctagaaacaaaaatcatagtgatgagcagtgctggaaggctggtcagcagctagagtacagcttgtgagcagcatattgggatttttttttttccatgttagactctattccaactctttctattgagagtccacggttttgtgatgggttgttgatgaaggaaagctctgaattttttagagcggatgaagtgtttgtcattttattccattttatgttaggttaacactgccatttttcttttattattcgatgtcttagctgatgtctcccaggcgaaaagtacccagaaaatcatgagagtgcagttcctggaaattcagttatttctttctcgctgggcttgctctgcctttagaattgttgtgactctggattcctgcggaggaactagggcctggggtgacctcatggctcctcagctatgatgcaccttctcttttcttcccttatctcaagtaggtcctgagcagcccagcccaggtggtctcttctgctcaccaggggtggcctggagtcaattgataagagccctcttttcttggcccttacaaaacaaatttctgcctaaagacagctaaagggaagaaaaacaccaccaaaccaacaactcctttgtacctccattatccccaaaattagataaagaaaaattagaataccaggaggcagcagacacctccacaatgcagctcggaaacagaatttctatagatctgctgtcctttttttaaaatcacatagaagagtttgtacaaatctcatttgttttcacttccttcatttttgtgtcttaacacattattttgaggaaaatgcctctgaattttatccttgctcttcaattacggttgaacaggaactgttaattgagtttagccactcaaaagaagaacaaagtatttcatcattcttacatattctggttggactcatggttaaagaagacaaatagaaaaactcacacatcagcctggtgtggggataaaaccaaaaacagtgatgctcacaggcatgcctgagagtggaatggtggtgttggtgggggagtgcctgtttactggtagtaggagtaactctcgtcatcatattccagctcatctatgtcatcgtcatccagcagcccatatttaaatttccggtagactgtgccatcctggcccatgtagacgatgtcatcatcatcatcctcatcatagtcccgatccctgtactcaatcacctgatcctcttcaaagctggtgctctctctatagctgctcttataggaggagtaagacttgttggggtcggccagtttttcatagccggcctttgctgctggctggactcggccacgagatttcttccacactaccacagctgccccgagcagaagcaccagcatcatggaggaggtgatgaacagagctgtcttgaaatgctcagttgcaggcctaaccttgcttgttcgaaggatgcattcgtccgtggtgtcctggcagtcacagcactcctgggcactggggggatcagaggtgttgcagcagtggaggcagtggctgtcgtccatgtgcagcaccaggttggcagggcacaaggtgcagttcttggcccctggtcccttgcattccatgcagctctcgtggcatttttcacagttaaacttctctccctctcccactctgtattcccccacaagacagtccgaggtgcagatccctcccatgaggtggtaactccacacacaggataaacaattcaacgctccttttcctttgcattgatcacaagtcggatggcatctctcacaggtctgtgtgctttgctctacatagtaatggtctgggcaggagcgatgacactctcctttggagcggagcagaaagaaaaatctatcgcaagacaggcagtctgtgggccgtgggccctggcaccccttgcagctcctgttgcacctctcacaccggccagtggagttgtctgcgtaatatccttccctgcactggagcaggcactcttttcctagctggaaccagcccggtcggcaggagtggcactgcctgctgtgtctcccttcacatgtcctgcaagagctgtggcagtgggcacaccggttgctgtcctcatcggcataatagccctctgggcagtccttcacacaggttgtgttgagaagaaggctgttcatggggcatgtttgacactggtcctccgccggccccatgcagtggaagcacttaacatggcagggcttgcacccgggagcatcctcatcccagtactcggagggtgagcacttctcgttggccatgcagctcccacgagggttcatgatcaggcctttctgacaggtggtgcaggtcccagatgatgagcaggtcaagcaggacttgtggcaatctctgcactccttagtctccttttcataataggttcctgctggacactcctccaagcacagtccatcatagaggacccaggaactctcaagacagagctcgcagtcgtcggctttggggccactgcactccagacagtctttatggcaggggacacagtggcgcgagtctgcatagaagccacggggacaggactggtggcacatatcatcgtgcaggaagaactcaggcgtgcactctttgcatgttttctcatggatgcagtcctgacacatctctgggcaatgcttgcatacccccttcacagccacgtgcctctcggggcagttttcctggcacactccgtggtgcaggacgtggcctccttcacaagaatggcagttggtggcgtttccttcacatgttctgcaaggagagctacagcgttcacatatgccgtcttctgcataagagccctccgggcacttggagtagcacctgccttcatggaggaagagagggtggcccggctgcatctggcattttttgcaaagatcggctccagagcagatggcacaggcctccgtacagttctcgcagctcccactccttacggaaggccatgtgccttggggacaggaggaaacacaggcctgagccagaagatatgcacctttgggacatgaagtgcacagagttgcagatccattgcaggttttacaagaagaatgacaaggctggagttttctcaaaatatcattccagaatttgccctcctcctgggtcttggtggcatgcacgcacatcccacgcagcagctgcagtccttcctggcagctgctgcactcgtcatgaccagggcctgtgcaggtttcgcatgctcggtggcaggactcacattctcccatttcttggtcaccatagaatccaggaccacatttcctcacacaactgccacctaagagaaagaagccctcttcacaccagtaacacccattctggtcacagctgccacagttactatcacacgccttgcattccacttcctcactgtaggtcttctcaggacaggttttataacaatggtgatcaaacctgtaataccccatagcgcaagatgtacatgttcctggatcatccaagctgcatcccagacatccttcttcacaagggacacattcttcatagtctgggtcttggacttcaccttgtccacactctaacttctggcatgtgtggttggtgggcgctatgaagtagcccttcatgcatcttgtgcagacatgcacgctgtggcaaagctcacagttgtctgggcagggcaggcaggtgttcccctcagtggcatagtggccctctgggcagctatctccacactctccctggtacaggaagtgctctcggccatagttgtctgctccacaggaggtgcagtgggtagggccacttccttggcatctctggcaggtgtggtggcatggatggcattggttctcaaattcaaatttccatgaggggcagttcgaaacacagcggccatcatcaaaaatccttgtcatggggcaggtagtgcagtcttcctgggttggtccctggcacttggcacatgaggcctcacaggtctggcagtggccatgctcatcaacatattctccatccttgcaaatggctcccatttgacacattcctaagtctaagagatacccactagggcagcttgtacagttcttgaatcctgggccattgcacgtcaaacaactgatatcacattttttgcaggatttgtatccattctctgaagagtggtcaaagtaatagctgatactacagctctgcacgcatctcccatcctccatgaagtagccctctgtgcagttaatgcacccatcagctcctgccccagcacaagtggcgcagaagcggtggcagggctggcagtcctggccgttgaaataccgtccatcttcacaggagacagagcaccgggatccctgcaggcttaacccatccctacattctgtacagttatggaattcagtacatgtcttgcagttttcactgcatttccggcaaagatttttcttggtatcctgatatgacccatcagggcagtgagtaacacagctgttggtttcttcattcagaaagtatccatatttgcaggacatgcattggtcaccatggctcccaaagcaggactcacagttgggggcacacttcctgcagcgcttcttgtcggcgtggtagtggccaggggggcagctggagacacagatcctggtattgtttttcagcttgtagtagtagtgcaaacagtcattgcagtggtctggtcctggcccgtcacagccaacctcactgcactcagggtcgcagggacctgcataatcctctgtgccatagtcgtctgtggggtcttcaactcggctatagcggaaccgttccactttcggaaattcattggttggtgaatatggctgcacggaggtgccgtagaggaccaaagaccattctttcaatttacctggagtcttaaagttccttagctgagagggagtatcataaacttcaaggacccagtcaccagcagctctttctccccagcaatgaatggtcatgaactcccagtttttgaatccttccatggagtgatcaaatagcctgttggccaaaagctgagacctagttccagagggcgaggtcaggtagatggccaggtctcctctcctggggtgggtgatggtgatgcgcacaacgacgtgctccaggtagttgacatggcggttggggttatccgagcagcctgaagctttgtagatggagcgcactgcactgttagggcggattgtcttgatttgtcggtctgtgctctccacacacacgtgctgccggggaacggtggtccacttctctgcctccatcaccatggcttctgcgtccatcagtccaaatccataaagatggctcaccttaaaaccagcagcattggttttccagtcattagcgttcaaatgtcccgcacgggaagtcctgacaataacatgctgtacgtctctccaggtcagaaacggattggcttccagggccagcgcaatgatgcctgcagccatgggggctgaggctgacgtcccagtgtggttgtccgtgcaacgctgcctcagatctgtagtgatgattttcttatcgtaggactccccgctgctgtaggttgtggccagcgtggatgaacactcttccaggtaccaaggtttctttccgctttctgcagtgctgctgatggagatggtgtagatgctgttggtgtagccatcacaggagcagtggtctttgctccttccaccatttccagatgcccaaacaaacacagagccgaggcctctccgccccattctaacgccgttttcaaaggcttgccgggtgaggggggctggtccgtccacagtcttgccatcatcatccgggccccagctggcgctgtaaatgtgcacgtgctgggggttgaagctaactgattttgcttcaaccatgtccgtgacatctccgtccagcattcgcactcctccgatcttggcgttgaaagcaattccgactgtgcagtgcgaattgtttgcagcggctgccacttctccagcacagcgagtcccatgcttgttctcgttgcttgcatcataacgaggcattgggtccaagtcattcccattcacgtcgcaacttgccagagcatcgtagttttgcatcagatctggatgggttctctcaattccgtcatccaggatagtgaccacaatgttctttcccgtgtagcctctcttccaggctccttcgatattcatgtcagactggcagggatgtgtattgtcactgcagtgcatataccacatgctgggccacttgggatcattgaaataggtagactgggcacgactgaagtcataatccctctttgtccgcttttttaccacttgctgttggatccattccacctttggttccattgaaatgaaactgtgggtccctctgctcgagataactgaccttttaatcgtcctgctatggtagaagtggtagtagtccttcagggcccctatctgtcctatgttgatgaatccgtacttgctggcgatacggttggcctccgggaagcccccggcgattttgactgcccagtggttggtgtagacgcgcgtccgacacacggggagcaggcagcccccgagcagcgccagcacgcacagcaggtccaaacgtcccgggcagcagcagcggctcccccagcccatggtcccggcgcctcgctgctccctcgctcgctggctggttccgcgcactaagggcgcgcacaactaacttctccggcctgcgccgcccggcgagcagccccgggccgccgcagctcgcagccccgggcgatcggcaggaggcggctagccccggcagggagcagagcagcgagccttacgccggctcctagaccatccctggggctgccgggacctgtgctcccagctctccggcccgtggggcgctcggcgatgctccccggctcggacgcaggaggaggctgagtggggcgggcgtcctccgcagttgggtttcgcccggcttggctcccggactctccgactcggtctcgctcctcccggggcccccgagcgcggcggagatgaccagcgggagcggtacaggcagcgaccgggcgccccctctgctggcccgggctccaaacgctcgcttgctcgctcccagcgctccctccggctccgagcagcgcgcgaggattctgagtggc

SEQ ID NO: 15859 - RNA, 8686 nt, Homo sapiens
  source 1..8686: mol_type = other RNA
gctgggattacaggcatgagccagcagtcctggcaaggagataattttatttatttatttatttagttagttagttagttacttattttttgagatggagtcttgctctgtcacccaggctggagtgcaatggtgccatctccgctcactgcaacctctgcctcccgggctcaagtgatttgcctgcctcagcctcctgagtagctgggattacaggtgtgcaccaacatgcccagatttttattgtatttttagtagaaatggggtttcaccatgttggctaagctggtatcaaactcctgacttcaggtgatctgcctgcctcagtctcccaaagtgctaggattagaggtatgagccaccacgcctggccaaggagataattttaaatgatcaaaatttttggaggcatatcatacatgtacatgtatgatctctgaaaactgttttaaagataaagtcagcaaagtacagcctgttggccaaatctgacccaccacctgttcttgtaatgctgtgaactgagaatagcttttgcatttttaaattttaaaaggttgaaaaaaatcaaaagaagaataaaattttataatatgtgaaaattacctgaatttcaaatgtcagtgtccataaataaggttttattgaagcacagctcacccatccgttatgtaccagctgcattcatgctataatagcagagctgagtggttatgacagagactttctggccaagaaagcctaatgtacttactagctggctctttccagagactgtttgtcaaccctgttttaagagctttcctctaaagaagcacaagcctttagtaaactgaagacttcttcataaagattttctgtgtcagtgatacattatgttaaaaaaagaaaatccatgaatttagtaaagataacattgatattatagactaaaacaataggcatgactttaattatatttaggatgcttattttcccaccttatttcagtagcatagttataagaacacacgctttagggtgatcattcttttttcttgaattttgttgagctttgcatgaccttggactagttacctaacctcttgtaagcctcaggtttcctacaagaacagaataatagcaataccaacctcatgggagtatggtaagtaccaaaatggataagtggggcatttttgggggggaattacttagcttgttatctggtagtaggtgtgcaatagattataattatcatcattctctgaaaatgtcatttttgctttctggtgctccatttctagtactgcctgtaaggtctattttgacaaggaaatctgtaagaccctgccaacatcattttgcatagcaagagcccttctctgtgttacaatctggacaaaaactgtcctcagttgcatgaatccaagaatacacttgacagaagaatggaaaaaaggaagcctaggaagtctagaaacaaaaatcatagtgatgagcagtgctggaaggctggtcagcagctagagtacagcttgtgagcagcatattgggatttttttttttccatgttagactctattccaactctttctattgagagtccacggttttgtgatgggttgttgatgaaggaaagctctgaattttttagagcggatgaagtgtttgtcattttattccattttatgttaggttaacactgccatttttcttttattattcgatgtcttagctgatgtctcccaggcgaaaagtacccagaaaatcatgagagtgcagttcctggaaattcagttatttctttctcgctgggcttgctctgcctttagaattgttgtgactctggattcctgcggaggaactagggcctggggtgacctcatggctcctcagctatgatgcaccttctcttttcttcccttatctcaagtaggtcctgagcagcccagcccaggtggtctcttctgctcaccaggggtggcctggagtcaattgataagagccctcttttcttggcccttacaaaacaaatttctgcctaaagacagctaaagggaagaaaaacaccaccaaaccaacaactcctttgtacctccattatccccaaaattagataaagaaaaattagaataccaggaggcagcagacacctccacaatgcagctcggaaacagaatttctatagatctgctgtcctttttttaaaatcacatagaagagtttgtacaaatctcatttgttttcacttccttcatttttgtgtcttaacacattattttgaggaaaatgcctctgaattttatccttgctcttcaattacggttgaacaggaactgttaattgagtttagccactcaaaagaagaacaaagtatttcatcattcttacatattctggttggactcatggttaaagaagacaaatagaaaaactcacacatcagcctggtgtggggataaaaccaaaaacagtgatgctcacaggcatgcctgagagtggaatggtggtgttggtgggggagtgcctgtttactggtagtaggagtaactctcgtcatcatattccagctcatctatgtcatcgtcatccagcagcccatatttaaatttccggtagactgtgccatcctggcccatgtagacgatgtcatcatcatcatcctcatcatagtcccgatccctgtactcaatcacctgatcctcttcaaagctggtgctctctctatagctgctcttataggaggagtaagacttgttggggtcggccagtttttcatagccggcctttgctgctggctggactcggccacgagatttcttccacactaccacagctgccccgagcagaagcaccagcatcatggaggaggtgatgaacagagctgtcttgaaatgctcagttgcaggcctaaccttgcttgttcgaaggatgcattcgtccgtggtgtcctggcagtcacagcactcctgggcactggggggatcagaggtgttgcagcagtggaggcagtggctgtcgtccatgtgcagcaccaggttggcagggcacaaggtgcagttcttggcccctggtcccttgcattccatgcagctctcgtggcatttttcacagttaaacttctctccctctcccactctgtattcccccacaagacagtccgaggtgcagatccctcccatgaggtggtaactccacacacaggataaacaattcaacgctccttttcctttgcattgatcacaagtcggatggcatctctcacaggtctgtgtgctttgctctacatagtaatggtctgggcaggagcgatgacactctcctttggagcggagcagaaagaaaaatctatcgcaagacaggcagtctgtgggccgtgggccctggcaccccttgcagctcctgttgcacctctcacaccggccagtggagttgtctgcgtaatatccttccctgcactggagcaggcactcttttcctagctggaaccagcccggtcggcaggagtggcactgcctgctgtgtctcccttcacatgtcctgcaagagctgtggcagtgggcacaccggttgctgtcctcatcggcataatagccctctgggcagtccttcacacaggttgtgttgagaagaaggctgttcatggggcatgtttgacactggtcctccgccggccccatgcagtggaagcacttaacatggcagggcttgcacccgggagcatcctcatcccagtactcggagggtgagcacttctcgttggccatgcagctcccacgagggttcatgatcaggcctttctgacaggtggtgcaggtcccagatgatgagcaggtcaagcaggacttgtggcaatctctgcactccttagtctccttttcataataggttcctgctggacactcctccaagcacagtccatcatagaggacccaggaactctcaagacagagctcgcagtcgtcggctttggggccactgcactccagacagtctttatggcaggggacacagtggcgcgagtctgcatagaagccacggggacaggactggtggcacatatcatcgtgcaggaagaactcaggcgtgcactctttgcatgttttctcatggatgcagtcctgacacatctctgggcaatgcttgcatacccccttcacagccacgtgcctctcggggcagttttcctggcacactccgtggtgcaggacgtggcctccttcacaagaatggcagttggtggcgtttccttcacatgttctgcaaggagagctacagcgttcacatatgccgtcttctgcataagagccctccgggcacttggagtagcacctgccttcatggaggaagagagggtggcccggctgcatctggcattttttgcaaagatcggctccagagcagatggcacaggcctccgtacagttctcgcagctcccactccttacggaaggccatgtgccttggggacaggaggaaacacaggcctgagccagaagatatgcacctttgggacatgaagtgcacagagttgcagatccattgcaggttttacaagaagaatgacaaggctggagttttctcaaaatatctcttttgatttgaactttccaccttcgtcgctcctgcagcaggctcttcaccacagataggtttgcagtggacacagcttcattccagaatttgccctcctcctgggtcttggtggcatgcacgcacatcccacgcagcagctgcagtccttcctggcagctgctgcactcgtcatgaccagggcctgtgcaggtttcgcatgctcggtggcaggactcacattctcccatttcttggtcaccatagaatccaggaccacatttcctcacacaactgccacctaagagaaagaagccctcttcacaccagtaacacccattctggtcacagctgccacagttactatcacacgccttgcattccacttcctcactgtaggtcttctcaggacaggttttataacaatggtgatcaaacctgtaataccccatagcgcaagatgtacatgttcctggatcatccaagctgcatcccagacatccttcttcacaagggacacattcttcatagtctgggtcttggacttcaccttgtccacactctaacttctggcatgtgtggttggtgggcgctatgaagtagcccttcatgcatcttgtgcagacatgcacgctgtggcaaagctcacagttgtctgggcagggcaggcaggtgttcccctcagtggcatagtggccctctgggcagctatctccacactctccctggtacaggaagtgctctcggccatagttgtctgctccacaggaggtgcagtgggtagggccacttccttggcatctctggcaggtgtggtggcatggatggcattggttctcaaattcaaatttccatgaggggcagttcgaaacacagcggccatcatcaaaaatccttgtcatggggcaggtagtgcagtcttcctgggttggtccctggcacttggcacatgaggcctcacaggtctggcagtggccatgctcatcaacatattctccatccttgcaaatggctcccatttgacacattcctaagtctaagagatacccactagggcagcttgtacagttcttgaatcctgggccattgcacgtcaaacaactgatatcacattttttgcaggatttgtatccattctctgaagagtggtcaaagtaatagctgatactacagctctgcacgcatctcccatcctccatgaagtagccctctgtgcagttaatgcacccatcagctcctgccccagcacaagtggcgcagaagcggtggcagggctggcagtcctggccgttgaaataccgtccatcttcacaggagacagagcaccgggatccctgcaggcttaacccatccctacattctgtacagttatggaattcagtacatgtcttgcagttttcactgcatttccggcaaagatttttcttggtatcctgatatgacccatcagggcagtgagtaacacagctgttggtttcttcattcagaaagtatccatatttgcaggacatgcattggtcaccatggctcccaaagcaggactcacagttgggggcacacttcctgcagcgcttcttgtcggcgtggtagtggccaggggggcagctggagacacagatcctggtattgtttttcagcttgtagtagtagtgcaaacagtcattgcagtggtctggtcctggcccgtcacagccaacctcactgcactcagggtcgcagggacctgcataatcctctgtgccatagtcgtctgtggggtcttcaactcggctatagcggaaccgttccactttcggaaattcattggttggtgaatatggctgcacggaggtgccgtagaggaccaaagaccattctttcaatttacctggagtcttaaagttccttagctgagagggagtatcataaacttcaaggacccagtcaccagcagctctttctccccagcaatgaatggtcatgaactcccagtttttgaatccttccatggagtgatcaaatagcctgttggccaaaagctgagacctagttccagagggcgaggtcaggtagatggccaggtctcctctcctggggtgggtgatggtgatgcgcacaacgacgtgctccaggtagttgacatggcggttggggttatccgagcagcctgaagctttgtagatggagcgcactgcactgttagggcggattgtcttgatttgtcggtctgtgctctccacacacacgtgctgccggggaacggtggtccacttctctgcctccatcaccatggcttctgcgtccatcagtccaaatccataaagatggctcaccttaaaaccagcagcattggttttccagtcattagcgttcaaatgtcccgcacgggaagtcctgacaataacatgctgtacgtctctccaggtcagaaacggattggcttccagggccagcgcaatgatgcctgcagccatgggggctgaggctgacgtcccagtgtggttgtccgtgcaacgctgcctcagatctgtagtgatgattttcttatcgtaggactccccgctgctgtaggttgtggccagcgtggatgaacactcttccaggtaccaaggtttctttccgctttctgcagtgctgctgatggagatggtgtagatgctgttggtgtagccatcacaggagcagtggtctttgctccttccaccatttccagatgcccaaacaaacacagagccgaggcctctccgccccattctaacgccgttttcaaaggcttgccgggtgaggggggctggtccgtccacagtcttgccatcatcatccgggccccagctggcgctgtaaatgtgcacgtgctgggggttgaagctaactgattttgcttcaaccatgtccgtgacatctccgtccagcattcgcactcctccgatcttggcgttgaaagcaattccgactgtgcagtgcgaattgtttgcagcggctgccacttctccagcacagcgagtcccatgcttgttctcgttgcttgcatcataacgaggcattgggtccaagtcattcccattcacgtcgcaacttgccagagcatcgtagttttgcatcagatctggatgggttctctcaattccgtcatccaggatagtgaccacaatgttctttcccgtgtagcctctcttccaggctccttcgatattcatgtcagactggcagggatgtgtattgtcactgcagtgcatataccacatgctgggccacttgggatcattgaaataggtagactgggcacgactgaagtcataatccctctttgtccgcttttttaccacttgctgttggatccattccacctttggttccattgaaatgaaactgtgggtccctctgctcgagataactgaccttttaatcgtcctgctatggtagaagtggtagtagtccttcagggcccctatctgtcctatgttgatgaatccgtacttgctggcgatacggttggcctccgggaagcccccggcgattttgactgcccagtggttggtgtagacgcgcgtccgacacacggggagcaggcagcccccgagcagcgccagcacgcacagcaggtccaaacgtcccgggcagcagcagcggctcccccagcccatggtcccggcgcctcgctgctccctcgctcgctggctggttccgcgcactaagggcgcgcacaactaacttctccggcctgcgccgcccggcgagcagccccgggccgccgcagctcgcagccccgggcgatcggcaggaggcggctagccccggcagggagcagagcagcgagccttacgccggctcctagaccatccctggggctgccgggacctgtgctcccagctctccggcccgtggggcgctcggcgatgctccccggctcggacgcaggaggaggctgagtggggcgggcgtcctccgcagttgggtttcgcccggcttggctcccggactctccgactcggtctcgctcctcccggggcccccgagcgcggcggagatgaccagcgggagcggtacaggcagcgaccgggcgccccctctgctggcccgggctccaaacgctcgcttgctcgctcccagcgctccctccggctccgagcagcgcgcgaggattctgagtggc

SEQ ID NO: 15860 - RNA, 6388 nt, Homo sapiens
  source 1..6388: mol_type = other RNA
gctgggattacaggcatgagccagcatgcctggctctccagatagttttttatttacactgatgtttccctaatgaccctacaatcagctacaggagggagattttgtcttcagcaaagaaggattgtcttagagcaccatgaaaaacgtcactacctcaggtacttcaaagactaggctcctgaacacaggcttctcatgacatcacatcaccacatttaagataatggttagtggacagagtcagaatttccagaacaccttaactgagacaaatttgtgttcataacacagtttaatacaatgtccagtggaacaaaatctaagtttgcaaagtccaaagacctatactataaaatcagcacttttctcctgacctgtctggccttacccaaataaagcacaagtgaatattcttgggagtgagttattgagtgcttcccaagaaatccaagagaccctaacaccttggtattgaagactttagcttctttttctcagaggagaacattaaacactttctcttttgagacccctttttcaggatacaatagaggaaagagccccaataacaggtaaggaaggccaggccatcattctactgtgctgcccactcaccatgtgactttataagagctgattactatcactgggcctcagtggcctcagctgtaaaatggagaccctgtactctgaaccctatttacccattttccatagaactattttgttaggaaaagagcacagtcataagtacacatctctagctgagttttgaaataatttttccatttttctcactggaaactgatgggtccccaagtaaactacactgtaggagaccagaacccagttctgcctctcctttcatgaagactccctttcacagttgccttggtgaattctttttatcctacatttcagaactcaacaatctcacatctgccgcatctaacatgccccactgatgctaattggtttccttaatatcttttgctttaacagaagtagttcagcaacattttcaccagtattatgctaaagtcctaaatataagaaggataaatctgttttcatgaagactctgaaggagaaacaataccaactgtaggtcctgtttactgcttttcattagatttaaaatctaaatctaaatctaaaaagtttgaggactggtacaatgaaatatctgttaccagtcagttatgataagtatggacattgagagctggcatttaggaatctgtatagcatctgatttagccacaacatttaaattagtgggctcactttttgaacaaggtatataccagtgcagttgttaaactcaaatgacaagtcaaatatgagtggcatactagtaatacaaccacatatcagttcacaatttactggaacaagaaaaacaaggaagtttgctactactggtcctaccccaatgatattttgagaagcaatgcacaatatactacttcattaaatgagattgattgttctgagtactgtgaacttagaattaacttgtagtgagagtaacaaactcaagtatctctattaatcagacaactactataaattaatgaagtgaatcagatatgggactttatagggaagagtgtggaaggaatgtggcaaaccagaggcccagtcttcatggtgcagtagctagtcatctctatgtgactgtaatcatgtgtaccctcctttttacttctcaagagagccagaaatccagactttcaggtaaaatgttattgattttcaaatgctaccagctcattaattttcttttaagatgtctgcttagaactagcaaacctatctgccatccagattgagttgtaagatgccactttgtagactgcgctttaggaaataatatattagagattagtactgtcagggttgtccttagggccatgtggaagatgtgcttgtctaaatcccagaagtctttcttgccatatcatgtccactgaacctcatatttccaggcacctcattgtcaagctgcccaccccaccactgcatgattccttagggagcgccgtggagcactcccagccttagcccagctgctcgcttcctcttctgtgcatttgagctgcaagcaggcctctctccagcagcttcaggtggggagtctccttcagctcatcacttcatggcaacagcagcaccccctcccctggccgaagtgaaacatctttgtgtccaggacatgggtttctcacagcccagtttttaaacacataaccgctatttccttcattctcaggacactcctgtgaattagccaaaggccaagctgggtccttctgcttagacagaggcagagagagggcgagtcacaaggcaggaggagaaaaagggacaccagagtggggactgcctggctcgtgtccctcttccgctgtctccttcctctgctgggcactctcctgtctctccatagggctcagcaggatgtcactctcacagccagtggcccaagtgcccaacagtaacctgagaaccagacccagatgtaccctggggaagcctgcctgcgtgtctggggttaggggaggagacagatgcagctgcttattaagggccacactgtgcatatccaaagtggactcaatctttgggaaaactaaagatagagggactctctgctattttacacatgagcaaacctgcccagcaggagtaaatgaaagtccaagatcacatggccagaaagtggtgaactaggatctcaaacccaggttgtctgatctgttattgaatctggctgggcagcatctggccaacaggcagcagaatgtggccacagaggatccaaggaacaggtgaaaacctaaaatatggacattcacaggcaaggggacagattgctacaacacttgatgtgacaccttttttaaacagtacagagcacaagtttttaaaagtacagtacatgctttagaggccatcactcaagacagaattacataggttatttctataccttttgaacctgtttttggccattgataactctatgctgttctatgaaatacatgatcatacacagattattttttctgggaatgcgattgataattgtgtttataatggaatacatttacaaataagttttgtaatattttgtaaccattaagaactgattggattgcatgtcctaggccagagagcttttatataatgttactacttaatttaacagtgtccacaagaggacagaagaatatattccaaacaatgtgtcatagtaccagttactaatccctgtctcaagtcctcttttggaatgaggcagggtacaaataaataaataaaataacatgaccataacttttttttttgcattttttccttatgttttccccatcactcctcaatctccatgtaaagcctgtcccatgaagttcatgccagctagtatgcagtgtgccccctctccacccatccctgtggctactgccctctgacttcagacctttgctattctgaataaagcctcccgcacctcagtcagagtctgcagctccaccctaggtcccagcatcaggttaggaatttatcaagcctaggaggctcccagcaactacctggcctcacaaggccttccagttcaaagccaatgaggaagtctctatatctttatccccagtcagctcctcccgccagggccagtgctctcaccaaccactggaaactgccccttctaaaatcactgattcaaacaccccacactggcaacaccttccacccattcagctctctatgggatagcttctcctggatgtctcaaggacacctccaacccaaaatgagagaacctgagagaagtcaggggcactgtcattaaagactttaatagcatgggctgatggcagcagcctggggtctctcatctatgggaatttttgaggctggatgaaattgttgatgaagtcctgccaggttctcagacccaagcatccctccttctcgggctggggcacctcatcaacctgatggtgggtacatcctccaagaggcatctgagctgcttatccttgtgcatggccctctctatgtgttctggtgtgatgcgcaccctgcaattgttctgggccttcttgcctgcctgctccaggatgttggccatcagatactagagaataacaaccaggaaaacaggtgtggatgagctcaggcactgggcatactgacctcgcagaaagccgtccatgtggctaacaggaaactgcagctaggcttttgtggagcagggaagaatctcctttctaaggctcctttttgccttcacatggtcttggtgagttttgttttgatcagccctcgtcgattttcccactagcctgagcctctccaggtaccagtgcttattcccgcccactgtgctccaggccctccttggtcagggagctgccttcaagacaacctcaactttgtgatattattggtgttcactgagccctgatcaagcccggcctcaaaatgtttctgacaggaacctgctcaccctaataactggaccgtctttttgaggaaagtctaactttgtacttgacttaaacattctagcaacaacaaaaaaaatgtgtttcaatcaaaacattgtcctgtcttcagtataccaatccaggttctctgattctagctttgtattgccagtgagctcatttacattcttctgtaagctataagtcactaacagacatgctcaatgtcttgtacagtagaggttcaaatgtcacccccccatgctgtaataaaaccagttttacttccatttacatattcattttgatatctctagtcaatattcctatgtctgtcctttgggttatcttataagctggtccgaagagaacatctgcttgttctctcatgagttaaatagaatctttaaaatgtattcatttctttaagtctggaactgaaagtaaaatatacctcgcaaacctgtcactaccaagacaaatggagatccatggctacagcagtccatatcaggaactgggaattattcttgacatctctcactgcctcaccttcatatccaatcaatcatcacattgttccacttacgcattcttaatattgctccaataatccactctgactattccagtccaggccattattctcaccttgacaactatagtagcccacttcctagcctctccatttgtttcttcactctcttcaaatacattttgcagagtaatcagtttctaaaactaaatttgatcatgacacttgttgcttaaaactcatcagtgccttcccattgcctctggaataaagcttgaaatcctgggatgctctttcctgatttttcttcacctggcttcttttcttcatctagcagttttcagtttaaatctaagttttggaaacatttgcctcatttcccagactcggttagacaacccccaatataccctcagagaggctacttatctttcactttgcaggatttaccttaaataaaatatgcatttgattaataatttgtgtgatgtttatatatcctatttgaagatgattggggcctgcctaccttattcaccactttatcctcagagaccagcacagggtttcttccaacagtgacgtcctgctgcatgacacttatgtacagctgtagggtcagctggggggctgagcccaagaaagcctggatcaccgacgcccggctgaacgctgatcggtgggtgattagtttgccttctgcctggcccacctccttctcaatctcctctgagaggccattttttggcatttgcctcttcttggtgatactgacataaggctcttcattgttgcctgactgaaagtagatgcagaagacttcaaaacacctgaaaaggggcccaagttgcagcaggtgcagcagcagtacgagcgggcggtcgcggctgaggtcgcggtgtacgaagagaagcgtgagctgcacgagcgcgcaaggcagtagcgagaaaagcaacgtcagcgcctgccacatgcggtccccgcccgagcggtaggtgctgctcaggctgagcgccgccgttgtctcggccacgaacaggaacacggacgccagcaccgaggccgggaatttcatctccgcgcgtcagcggcgctcaccggggacggacgcagtggcggcggctgtgtggctgtggcggcggcggccgttgcccgaggggctcccagcatgcccagccccaaaccgctcccgcgctctgcgcagcccgccgagggcacgcgggcccggccgaccggcctgggctctggaactggacctggtgggggcggccgacctggctggggtggggtggggtggggcgagctgcgcagccccgccgggacacgcccacgcgctccgtgcgccgcctgc

SEQ ID NO: 15861 - RNA, 7234 nt, Homo sapiens
  source 1..7234: mol_type = other RNA
gctgggattacaggcatgagccagccaaattctagttaaattctatggttcatgcagaaatgggttactctacccattttgagcttatttccatttctcccatttacatgccagagttttagaatggcaatactgggatgctatgttaacttctattttagataaatcagacttcttatttagggggttatttggtaaaattagaccaacagaaaattgactgtgacttaaatattcttttaaattcatcccaaagttacactatgcagtgggtccactagactcattttcttatgttctattttgacattcctagtgttttatacacaattagtgtgtgatatcagtattagctttttctgtatgaaatactagtctcaaaattaagtggtttaaaataaccattgacttagctcatgatttcatggcaatttttcctaaatttttttctagactatttattcatattaaagttgttcatattccatataaagtatatgaagttttagaaactacatatttcttaaaatgttacagcaaatgaaaataatactgtattttggaatatgggttatctaccctcagggtagataaaagtaaaaaactagtgttgaaatgcaatgtaccagcccatagcactgaacaaaatgaactttcacttaccagtatttacattgtacctattcttaatataaaccactcattatatagaaaagtgctttttgttaggttttttaactacatagccagttaaaaattattttttcccactatggacaagaaagggaaaatgaagttagcatataacaagagatacctggttgggttggatgaccagcgtaacagagcctcaaatttatcttctgttcttatgccttcccagccctggcccctgttccctgacactggcctgtggaatctctggactacaggataacttaacatctcatctactggttaaatctagcaggcatcggaatcccctgggaaaactcacaaggcccacctgcagattgatttggctgctcaggagtggggattgggaatgtgcacatttaataaggttcccaggaggttttgacatgtccattcccactctagttcttacagtggagtctggttcctgtggtctagtgcagccacttatcggatgcaggggtcccacctcagcttctctaagtggtcacccaggtgggatgctcactatcttctgaggcttattctgtttttcctttttttttttttttttttttggtttgtttttagctactctatactatattcagatttctgtcatttttacctaatgttctttttctgttcctggatcccatcctggatcaggtggtatgcattcttataagtgaaatattaatatatcaaaattactcattttggcaaatcagtatattttctgtatataattatagaaagttcacattgttcttcaaatttacttgtaaaaaattattttccatttggcactaaagtttattctcaaggtgttcaatctatgtcagtttttatttgaagttgtgtgatctctctaaaataaacattagtaattacttacaaaatgctccttagaatctcaatctggtttattgttttaaatcgcaatgttatacttatgtgcaaaaatatacttaaggtatattatggttgtaggttaacaattgcattggcaagattcatttttcctgtatgtttttactgaatgatctattttccaacccaaggaaagtatgaatatgtggcatgatgacacaacacctttcctagaaatgtgtttactgactactgagtgtgcctttggtaatcctgttaaaagcaatggaaaaataaaacatgaccaaaaataagaaaaggaataagccttgtcttctggggattaaagctgaatggaccacatacccacaaatgcacacattagaggtcagtactatcactaccattatctcagtgaaaaatgaaagctggaagaatttaatcgtcaagactgtgatcactggggtctaactcgacttcaaatcccaactctgctctcaccagcagcttatccttgggcagatgattcaattgctttaaacttcagttatttcaactaaaaaatgaggagacaattctatctcacagaataatgagataaggcatatgaagcaattagtatagccctgccatgtaatactgagcccctacatcatgttgactgttattataatatatacccagctgaaaactcaataatacaaatgagctggggaacatctaaaactatcatatggagaatgatttttgctaactccagcaaaaagcaaggctgtatgaccctttatttggcaatgttaaccatacttttcttctttttgtcctatagccccactctcaataactgccatctacattctctcttctcctctcagaaatctcactctgaataacttaatgaccatagtactcacacttttttaattaaagtgatgtgtcctcacaaatacatttctcaaactcaaaacatcatgcttgaaatatcactgaacttgtcaccaaagaagtcacatggcaatgataataaagaaatatgcagactacactctgaggatagagctctaaagagtaaaaacaatggaatttggaaaaaataggagtaaagaattgctttgagcaataaaaactgagattgataagccacttttctttttgatataggcttgtcactcacagccaaaatctctcagcaaaaccacagctactgtttaccctcctgagagatgctccttcctcacccaacacgcatcaaccttcctagaaaggtttatcctctttacaattcttgttaaggtggcactgaatacaaagttactcatgatcaacttccttactagttgtcagtgtctgcccttctagaatttcatgtttgtgtcaaaattatttattgagttccttataaacatggtcatatctatgcagagtgctgtggagtttataaagacgagtaagatgatacacttttgccttccagttagcagagttaagttgatgctattgggatcatatgccccccaaagctgaagatatttactttcttagcccattaaagaaaaagtatgccaaatcctgaaataggagatgcaagtgtaggagttcacacggaagaaaggtcagtttcaacaagggtaattcagagaaaagttttggaggaagtttcaatagaaatagaactacaagaatgagcatacagagggctaaaaatgtctgactaataacaaaaaagacataaacatgtgaagaaaagaaaaagaaaggtagacgatggagcctgcccatttagtttatatataagctctcttaagatgatgtacaaaggtattttcatttttaccatttttctaatcagcaggtatgttttatacaaactatattccatatgcctctagagtgtctcttaattacatgcttgccctctcgccggtaaccccactctgaagaggcaagcccagggctaagaatttgagacaaataacacgttatcattaacggcattctctgaaactgtgccacaattttaccttcatcttctctgtcacttgatttctaatatttattcagcaccaaaacaattctttttcttccaagaccaagtcatatgactatgtaacatattaagttgcaaaagattattaccatattgttcatatcatttgtatatttgtatttgttctttttccccaaagttccagtaaaaaagctagagggattagttctagtcttaaaagacaaaaaaaattttgcttaattcagaaagaatatattacattaacaggtctaggtgagctatttcaaagagctttttgttcctcaactcctttataacatcaaaaagcttttgaaatctaaatttgcatccaaaaaatttattgcagaaagacaatttacattgtcttacatgaatatgtaaaaatatcttatgctcaatactaaaactggtggtcatatgaccttttggccagttatctaaatagccacattttcatattctactttacacacttacaagctagaagaactattaactgtagtttacaaaaaattaattatttgtaagagaaaatgagtatcttctaaaaatataagcaattcttgaactgcagaagaatgagccatcacatgtaaaacttgaagaaaaattttaagtagaactttaaacatgtaaattaggcaaaaacaaacaacacacaaaagtgagtgggagaagagagaggaaagaaggaacaaacaaaaacttgtaaactgtgacaatctaaattcaggttactgctgtcctgatatgaagatataagaggaaaaaataacattttaaactcaaaaactaaaatgttttactatttcaacatattacttcctccagaactctcataacatgtacataaataagaatgtttctcatttcttaatttattaacaatgtatacatttgaaaaaatatatacaatatttcaaaacaagcccttcaagactatatttaagcaatgacatccaaggaagcagaactcaggtaccatgtaatatttggaaaatatggtaacttgaagattaagatttctcttccttgctggttactctgaagtctccaatatacaaaggttgctcctaacgtggttttcttattgagccaagcatcttgatgggtcaatcccagtttcattttctccagtactgggcaaacttgtgaatctgttccaccactgcagcaaaaagagcatggacactctcatcaatcagactctgcatgtaatgcacagcctcttcatccgacaggtctaagcggaatttatcctgaacctttttcacagttttatctggttcaagtgcaatatctggaatgtttgcatcaaccatcaaggaaaacaagttcaaaatcagattagaataccttcgcaggtggaggaaagccgtgtaacactgtttacggaactcttggtactgctcactctgtgtgccccccattccttctaccatttctttattcagcttcattggtggaggaagaggctttggatcccgacccaaaatatatccaaagtctatgtggaagagtttgcctgtttttgttagcaaaaggttatccaggtgcctgtctccaactccaagtatataggtgatcacgcaatatccagcacagcttttaacgtaagtgtccatgacctcagcactaatcccatttggcccattctcacttggtgcatattttctaaaaaagttctgaatgcttccctctgtatcaagaacttcagccacaggaactgactggataaactgcatgaagccatgttttgtactggtggctaacaccttataaggtgtcaatttcaagtccagattttctttccgtaacagcttgtccatgagtgaaatgatttgaagaataagttgatcttgacgtaaatcatctccatgcttaaatataactggatatttgcctccatcttccgtcttaaaaaacaactgtgcaggcataagggcacttttaaacagtgtagctgtttccggaattattcctctaattttcacttggggttctaaaggcaacgggataagttccacatctgacaaattcatcttttcattatctccaagcaatgcctgtagtctctcattctttttcttacgatttccactttcgcgttgtactgccttcattagatgcaccaaccgatctacaaatgtctgttgtgcagccagcaaagaacgcataactctgacagacttatcacccttcaacaatgcttggctgaatcttctcattacgttcaagtacatctcatgggtctttggatctctctgctgagtatcttgatcttcacattccactatcacataccagtataaataattagccagtgttgagtttttgcaggctctcgatatcaagaaggtacagagatcttgttccagattttcgccatctggaacttcttttgtttttgatgcaggaggaggtgaagagactgaaggaagggggctggttataatttgggagctatctatttctgcagaatttattccagaatttgacacattttctgacactgaactctgactatccttcttggtaggttccaatccattctttatatcatcaaaattttcatatttgagagcctggaccaattgtaataggtacatcaacaaatcctcatcatcggcctgtcgcaaccgggcaacagcataacgcctcacagttgggttggtgtaatgagaggataacagctccaaggagtcctctacatccatcggcttccattttcccagaagttccaaggcctgtttggcctcttgaggtagatcccaattaacacatttcaagaattttgtcaaggctttttcttgattcgtaagataatatctaaacttccaaacaagatcttgttcttcatatgtaagttgcttggttggtggataactcacaataatatttaactgatctctcgtggcagcattgggtttcagatcgtggtcagaaggtccacttcttaaactccgggcaagcttgtggtgtttgctctcaactaaattctccatagacatctgggggtcaggaactttcactaattcaaaacttgttaaaattggagatgattcatcaccgtccttttcataataaacaataccatattccttatcatcacacttgacacatcgaaattcaaccatcaggtacatgaaattagaacttcgtttttcactctcatttatcatttctatttctctaaatgtcaatctatccagccaatctactttcaccatgtgtccttgtcgatgagctttggtgagcttggcaagacggctcatctgatcttctgagagagtgctacttgttctgccaggagtttttgtgggttctgatccatctgcttctacattaggccagactttcaagtcatgcatcccttggcgaaacatgccgtattttccaaagagcgaaaccgttgttcctcctacaggcactgcttttccgggaccatacacatcccatatggtgagggccacttgggcattcctgggcaggtcagggtattttactggtagtttcagccattcattccagatcttaagctggacgttgatatccaggtcacaactatagatgtagtgaaacttctctgcttcccccatcgcaccgtctgcaaaggtaccacctacagcgggaacttaggtacaggaaaaacaacat

SEQ ID NO: 15862 - RNA, 7423 nt, Homo sapiens
  source 1..7423: mol_type = other RNA
gctgggattacaggcatgagccagccaaattctagttaaattctatggttcatgcagaaatgggttactctacccattttgagcttatttccatttctcccatttacatgccagagttttagaatggcaatactgggatgctatgttaacttctattttagataaatcagacttcttatttagggggttatttggtaaaattagaccaacagaaaattgactgtgacttaaatattcttttaaattcatcccaaagttacactatgcagtgggtccactagactcattttcttatgttctattttgacattcctagtgttttatacacaattagtgtgtgatatcagtattagctttttctgtatgaaatactagtctcaaaattaagtggtttaaaataaccattgacttagctcatgatttcatggcaatttttcctaaatttttttctagactatttattcatattaaagttgttcatattccatataaagtatatgaagttttagaaactacatatttcttaaaatgttacagcaaatgaaaataatactgtattttggaatatgggttatctaccctcagggtagataaaagtaaaaaactagtgttgaaatgcaatgtaccagcccatagcactgaacaaaatgaactttcacttaccagtatttacattgtacctattcttaatataaaccactcattatatagaaaagtgctttttgttaggttttttaactacatagccagttaaaaattattttttcccactatggacaagaaagggaaaatgaagttagcatataacaagagatacctggttgggttggatgaccagcgtaacagagcctcaaatttatcttctgttcttatgccttcccagccctggcccctgttccctgacactggcctgtggaatctctggactacaggataacttaacatctcatctactggttaaatctagcaggcatcggaatcccctgggaaaactcacaaggcccacctgcagattgatttggctgctcaggagtggggattgggaatgtgcacatttaataaggttcccaggaggttttgacatgtccattcccactctagttcttacagtggagtctggttcctgtggtctagtgcagccacttatcggatgcaggggtcccacctcagcttctctaagtggtcacccaggtgggatgctcactatcttctgaggcttattctgtttttcctttttttttttttttttttttggtttgtttttagctactctatactatattcagatttctgtcatttttacctaatgttctttttctgttcctggatcccatcctggatcaggtggtatgcattcttataagtgaaatattaatatatcaaaattactcattttggcaaatcagtatattttctgtatataattatagaaagttcacattgttcttcaaatttacttgtaaaaaattattttccatttggcactaaagtttattctcaaggtgttcaatctatgtcagtttttatttgaagttgtgtgatctctctaaaataaacattagtaattacttacaaaatgctccttagaatctcaatctggtttattgttttaaatcgcaatgttatacttatgtgcaaaaatatacttaaggtatattatggttgtaggttaacaattgcattggcaagattcatttttcctgtatgtttttactgaatgatctattttccaacccaaggaaagtatgaatatgtggcatgatgacacaacacctttcctagaaatgtgtttactgactactgagtgtgcctttggtaatcctgttaaaagcaatggaaaaataaaacatgaccaaaaataagaaaaggaataagccttgtcttctggggattaaagctgaatggaccacatacccacaaatgcacacattagaggtcagtactatcactaccattatctcagtgaaaaatgaaagctggaagaatttaatcgtcaagactgtgatcactggggtctaactcgacttcaaatcccaactctgctctcaccagcagcttatccttgggcagatgattcaattgctttaaacttcagttatttcaactaaaaaatgaggagacaattctatctcacagaataatgagataaggcatatgaagcaattagtatagccctgccatgtaatactgagcccctacatcatgttgactgttattataatatatacccagctgaaaactcaataatacaaatgagctggggaacatctaaaactatcatatggagaatgatttttgctaactccagcaaaaagcaaggctgtatgaccctttatttggcaatgttaaccatacttttcttctttttgtcctatagccccactctcaataactgccatctacattctctcttctcctctcagaaatctcactctgaataacttaatgaccatagtactcacacttttttaattaaagtgatgtgtcctcacaaatacatttctcaaactcaaaacatcatgcttgaaatatcactgaacttgtcaccaaagaagtcacatggcaatgataataaagaaatatgcagactacactctgaggatagagctctaaagagtaaaaacaatggaatttggaaaaaataggagtaaagaattgctttgagcaataaaaactgagattgataagccacttttctttttgatataggcttgtcactcacagccaaaatctctcagcaaaaccacagctactgtttaccctcctgagagatgctccttcctcacccaacacgcatcaaccttcctagaaaggtttatcctctttacaattcttgttaaggtggcactgaatacaaagttactcatgatcaacttccttactagttgtcagtgtctgcccttctagaatttcatgtttgtgtcaaaattatttattgagttccttataaacatggtcatatctatgcagagtgctgtggagtttataaagacgagtaagatgatacacttttgccttccagttagcagagttaagttgatgctattgggatcatatgccccccaaagctgaagatatttactttcttagcccattaaagaaaaagtatgccaaatcctgaaataggagatgcaagtgtaggagttcacacggaagaaaggtcagtttcaacaagggtaattcagagaaaagttttggaggaagtttcaatagaaatagaactacaagaatgagcatacagagggctaaaaatgtctgactaataacaaaaaagacataaacatgtgaagaaaagaaaaagaaaggtagacgatggagcctgcccatttagtttatatataagctctcttaagatgatgtacaaaggtattttcatttttaccatttttctaatcagcaggtatgttttatacaaactatattccatatgcctctagagtgtctcttaattacatgcttgccctctcgccggtaaccccactctgaagaggcaagcccagggctaagaatttgagacaaataacacgttatcattaacggcattctctgaaactgtgccacaattttaccttcatcttctctgtcacttgatttctaatatttattcagcaccaaaacaattctttttcttccaagaccaagtcatatgactatgtaacatattaagttgcaaaagattattaccatattgttcatatcatttgtatatttgtatttgttctttttccccaaagttccagtaaaaaagctagagggattagttctagtcttaaaagacaaaaaaaattttgcttaattcagaaagaatatattacattaacaggtctaggtgagctatttcaaagagctttttgttcctcaactcctttataacatcaaaaagcttttgaaatctaaatttgcatccaaaaaatttattgcagaaagacaatttacattgtcttacatgaatatgtaaaaatatcttatgctcaatactaaaactggtggtcatatgaccttttggccagttatctaaatagccacattttcatattctactttacacacttacaagctagaagaactattaactgtagtttacaaaaaattaattatttgtaagagaaaatgagtatcttctaaaaatataagcaattcttgaactgcagaagaatgagccatcacatgtaaaacttgaagaaaaattttaagtagaactttaaacatgtaaattaggcaaaaacaaacaacacacaaaagtgagtgggagaagagagaggaaagaaggaacaaacaaaaacttgtaaactgtgacaatctaaattcaggttactgctgtcctgatatgaagatataagaggaaaaaataacattttaaactcaaaaactaaaatgttttactatttcaacatattacttcctccagaactctcataacatgtacataaataagaatgtttctcatttcttaatttattaacaatgtatacatttgaaaaaatatatacaatatttcaaaacaagcccttcaagactatatttaagcaatgacatccaaggaagcagaactcaggtaccatgtaatatttggaaaatatggtaacttgaagattaagatttctcttccttgctggttactctgaagtctccaatatacaaaggttgctcctaacgtggttttcttattgagccaagcatcttgatgggtcaatcccagtttcattttctccagtactgggcaaacttgtgaatctgttccaccactgcagcaaaaagagcatggacactctcatcaatcagactctgcatgtaatgcacagcctcttcatccgacaggtctaagcggaatttatcctgaacctttttcacagttttatctggttcaagtgcaatatctggaatgtttgcatcaaccatcaaggaaaacaagttcaaaatcagattagaataccttcgcaggtggaggaaagccgtgtaacactgtttacggaactcttggtactgctcactctgtgtgccccccattccttctaccatttctttattcagcttcattggtggaggaagaggctttggatcccgacccaaaatatatccaaagtctatgtggaagagtttgcctgtttttgttagcaaaaggttatccaggtgcctgtctccaactccaagtatataggtgatcacgcaatatccagcacagcttttaacgtaagtgtccatgacctcagcactaatcccatttggcccattctcacttggtgcatattttctaaaaaagttctgaatgcttccctctgtatcaagaacttcagccacaggaactgactggataaactgcatgaagccatgttttgtactggtggctaacaccttataaggtgtcaatttcaagtccagattttctttccgtaacagcttgtccatgagtgaaatgatttgaagaataagttgatcttgacgtaaatcatctccatgcttaaatataactggatatttgcctccatcttccgtcttaaaaaacaactgtgcaggcataagggcacttttaaacagtgtagctgtttccggaattattcctctaattttcacttggggttctaaaggcaacgggataagttccacatctgacaaattcatcttttcattatctccaagcaatgcctgtagtctctcattctttttcttacgatttccactttcgcgttgtactgccttcattagatgcaccaaccgatctacaaatgtctgttgtgcagccagcaaagaacgcataactctgacagacttatcacccttcaacaatgcttggctgaatcttctcattacgttcaagtacatctcatgggtctttggatctctctgctgagtatcttgatcttcacattccactatcacataccagtataaataattagccagtgttgagtttttgcaggctctcgatatcaagaaggtacagagatcttgttccagattttcgccatctggaacttcttttgtttttgatgcaggaggaggtgaagagactgaaggaagggggctggttataatttgggagctatctatttctgcagaatttattccagaatttgacacattttctgacactgaactctgactatccttcttggtaggttccaatccattctttatatcatcaaaattttcatatttgagagcctggaccaattgtaataggtacatcaacaaatcctcatcatcggcctgtcgcaaccgggcaacagcataacgcctcacagttgggttggtgtaatgagaggataacagctccaaggagtcctctacatccatcggcttccattttcccagaagttccaaggcctgtttggcctcttgaggtagatcccaattaacacatttcaagaattttgtcaaggctttttcttgattcgtaagataatatctaaacttccaaacaagatcttgttcttcatatgtaagttgcttggttggtggataactcacaataatatttaactgatctctcgtggcagcattgggtttcagatcgtggtcagaaggtccacttcttaaactccgggcaagcttgtggtgtttgctctcaactaaattctccatagacatctgggggtcaggaactttcactaattcaaaacttgttaaaattggagatgattcatcaccgtccttttcataataaacaataccatattccttatcatcacacttgacacatcgaaattcaaccatcaggtacatgaaattagaacttcgtttttcactctcatttatcatttctatttctctaaatgtcaatctatccagccaatctactttcaccatgtgtccttgtcgatgagctttggtgagcttggcaagacggctcatctgatcttctgagagagtgctacttgttctgccaggagtttttgtgggttctgatccatctgcttctacattaggccagactttcaagtcatgcatcccttggcgaaacatgccgtattttccaaagagcgaaaccgttgttcctcctacaggcactgcttttccgggaccatacacatcccatatggtgagggccacttgggcattcctgggcaggtcagggtattttactggtagtttcagccattcattccagttccatcttgtactaaatgctttgtaggatgttctcactggcaaggccaaaggcttcccttctgcaaaaacttgacaagtaacataaagatcagagcatgtctcttgatatagtcctgagaacttcaacattgggtcttccaggacagctttataactcttttgttctctcttcccttccaagcttcctatcttaagctggacgttgatatccaggtcacaactatagatgtagtgaaacttctctgcttcccccatcgcaccgtctgcaaaggtaccacctacagcgggaacttaggtacaggaaaaacaacat

SEQ ID NO: 15863 - RNA, 2419 nt, Homo sapiens
  source 1..2419: mol_type = other RNA
gctgggattacaggcatgagccagcgtgcctgacctctctccttgattcttaacattgttctttggtcctcttattcctctgtccttttgctgggttttctctacctgctccttaaacgttggtgttctcttggcttcttttgctcttactaggcaagattatcagctggatgttccataggcacttcaaacttcacattctcttctccttgttttctgcataaaccctttactagctctccactgtttttcaccatcatgagggaaaatgagaactaatgtggactggcgggaggcagtctggggcggtaaccccgtatctgaaatactccagggatccatgtttctttcaatagtcagattaagcattccccaatccaatccccagatatctttgaacaaaatcaataaaaatcagtaaaaacaggaatatatatatatatatatatatatatatatatagacacacacacacacacacacacacatgcatatacacacacatgcatggaggaccatactaaggcctttttcaggtcaaaaagggttttcacattgaccttttttacttttaagtatttttcctcagaatgttccttcagttaaaaatcaggtttaatctggagctcttactgatttttctttgattcctactgaacacctagctactggccatggtttctttgaggaaaaaaacaccattgctgaagcatttctaaacatttttaatgcatgcagaaagaactacatagactctccaagcagctatataaggtggctcaagtaacattatgatttattttggtctaagccctttcataacgtccttttaaaatacaaagagaatggctacgaaatggtgccagaacccagaaggcccagctggactgacaggagctctgagcagttcataggacaagcagggacccgccgaacctctcccgtttctgtgctttctctaaatgcagcaggtcctctctttactgcccatgcttttaaactatgaaaaaaaattttttaaagaaatctagcagtgattaatggagacctcaaataacactgtacatgggctttgttagagacaggtaatcattcttaacagctcttttcccagaggaggcctgggtgggccgagaggcatccagagtttaggaagtgcttttattgcagactgcaccttggctaatactatcctctatgtactggctgcctgtgtcactcctgctgaggactgtggaggggatgcgagagggacgcctctctgggttctcctgagagaagcagcagatcatcttcttcatggtgccatacatgtcctcgtccttgtaggagtagatgatggggttcacgacggagttgagcagcgccagcagcaggaaccaccttttcacatgctgcacgccacactgcctgcagttcaggccgtcgaggagcagaaccaccaggcccggggtccagcataccacaaacgcccctaagacagtcatcaccgtcttcattagcttcatgggtgtcctccggcggctgatggacccacttgtatgcggagacaagacgttggttttcctcttgacgtacacgtagatccgcaggtacaccacaaccatgatgaggaaggccatgaggttggacactgtccagaaaacaaggtaactcctgctgtaaatgggggccagggaagagcaggcagagatgttgcagaggcaattccagcccagtgtggggaccgcccccataaaaatggcgatggcccagacaagcaaaatgagcagtgtcaccctctttttggtcaggttgctatggacccgcatcctcatgattgacatgtgcctctccacggcgataaccagcaagttggtgagggaagcagtcaagctactgtccagaagcccctgacggagaaaccagcggttgacagtcaaagtttttgaaactgggcctgtgttaaacatcaggaatacataggcaattccagcgaagaaatcggcagcagctaaattagccaacaggtagtagaaggggaaatgaaattttctgtttttgatcactgccgcgatgaccagagaattagaaaaaaaaataaacaggcagaaaaacgtcccaacacacaaaacaatcacaagctttgttcctgtccagtcatcgacagtatcagtgttgctcctattataaaaaaagtccatgtgcttgtcatagtgacactcattcattgtggagaagtgaacatccgctcacgttcacccgcgccgccgagcccgggagcgggggcccctgcggctgccgcatgccctcggggtcgagcgcgacggggcgaccgggcgccgggctccagccgggcgcggagaagcagcggaggacgcggcgggcgggcggagcgcctcctctccagcgacccctgcgacgcgtccagagccaaagg

SEQ ID NO: 15864 - RNA, 2912 nt, Homo sapiens
  source 1..2912: mol_type = other RNA
gctgggattacaggcatgagccagcgtgcctgacctctctccttgattcttaacattgttctttggtcctcttattcctctgtccttttgctgggttttctctacctgctccttaaacgttggtgttctcttggcttcttttgctcttactaggcaagattatcagctggatgttccataggcacttcaaacttcacattctcttctccttgttttctgcataaaccctttactagctctccactgtttttcaccatcatgagggaaaatgagaactaatgtggactggcgggaggcagtctggggcggtaaccccgtatctgaaatactccagggatccatgtttctttcaatagtcagattaagcattccccaatccaatccccagatatctttgaacaaaatcaataaaaatcagtaaaaacaggaatatatatatatatatatatatatatatatatagacacacacacacacacacacacacatgcatatacacacacatgcatggaggaccatactaaggcctttttcaggtcaaaaagggttttcacattgaccttttttacttttaagtatttttcctcagaatgttccttcagttaaaaatcaggtttaatctggagctcttactgatttttctttgattcctactgaacacctagctactggccatggtttctttgaggaaaaaaacaccattgctgaagcatttctaaacatttttaatgcatgcagaaagaactacatagactctccaagcagctatataaggtggctcaagtaacattatgatttattttggtctaagccctttcataacgtccttttaaaatacaaagagaatggctacgaaatggtgccagaacccagaaggcccagctggactgacaggagctctgagcagttcataggacaagcagggacccgccgaacctctcccgtttctgtgctttctctaaatgcagcaggtcctctctttactgcccatgcttttaaactatgaaaaaaaattttttaaagaaatctagcagtgattaatggagacctcaaataacactgtacatgggctttgttagagacaggtaatcattcttaacagctcttttcccagaggaggcctgggtgggccgagaggcatccagagtttaggaagtgcttttattgcagactgcaccttggctaatactatcctctatgtactggctgcctgtgtcactcctgctgaggactgtggaggggatgcgagagggacgcctctctgggttctcctgagagaagcagcagatcatcttcttcatggtgccatacatgtcctcgtccttgtaggagtagatgatggggttcacgacggagttgagcagcgccagcagcaggaaccaccttttcacatgctgcacgccacactgcctgcagttcaggccgtcgaggagcagaaccaccaggcccggggtccagcataccacaaacgcccctaagacagtcatcaccgtcttcattagcttcatgggtgtcctccggcggctgatggacccacttgtatgcggagacaagacgttggttttcctcttgacgtacacgtagatccgcaggtacaccacaaccatgatgaggaaggccatgaggttggacactgtccagaaaacaaggtaactcctgctgtaaatgggggccagggaagagcaggcagagatgttgcagaggcaattccagcccagtgtggggaccgcccccataaaaatggcgatggcccagacaagcaaaatgagcagtgtcaccctctttttggtcaggttgctatggacccgcatcctcatgattgacatgtgcctctccacggcgataaccagcaagttggtgagggaagcagtcaagctactgtccagaagcccctgacggagaaaccagcggttgacagtcaaagtttttgaaactgggcctgtgttaaacatcaggaatacataggcaattccagcgaagaaatcggcagcagctaaattagccaacaggtagtagaaggggaaatgaaattttctgtttttgatcactgccgcgatgaccagagaattagaaaaaaaaataaacaggcagaaaaacgtcccaacacacaaaacaatcacaagctttgttcctgtccagtcatcgacagtatcagtgttgctcctattataaaaaaagtccatgtgcttgtcatagtgacactcattcattgtggagaagtgaacatcctggtagcaatccatggaaagttaaccttgctgacattcctcttcacttccctctgttggatgttcctggaatttgcatttgtggaaagttgcatacttgcagtgaacaagttccactggtcctgttgtagtggattccacctaaccttttattcctctcatccctgtccagctaacgttctctcactgttcagcatatgtacgtcaaagacagaagtgcatgaagacatgtgtaaagatgcaaaattcccccaggaaactcattatctagagcagccagggccaatcctctcctcctcccagggattcctagcaatatctggagacatctgcatcagtcatgacttgggggaggggggtactattggcatctaccgggcagaggccaggaatgctgctgcacacgctacaatgcacaggccagctctccacaacagagaagtatccggtccaaaatgtcagtggtgctaaggttgagaaatcctgacctagagggtgagatgagacatataatacagggttaagtgtggcagagctgtaatagagctaaaactggagtgctatcagattgataacatttaaacaagcggctattacttgccaacaagtgttggcaagaatgtggggaaaatagtaccctcataacatgttggtgagaatgtaaactgatagaactttggggga

SEQ ID NO: 15865 - RNA, 2307 nt, Homo sapiens
  source 1..2307: mol_type = other RNA
gctgggattacaggcatgagccagcgtgcctgacctctctccttgattcttaacattgttctttggtcctcttattcctctgtccttttgctgggttttctctacctgctccttaaacgttggtgttctcttggcttcttttgctcttactaggcaagattatcagctggatgttccataggcacttcaaacttcacattctcttctccttgttttctgcataaaccctttactagctctccactgtttttcaccatcatgagggaaaatgagaactaatgtggactggcgggaggcagtctggggcggtaaccccgtatctgaaatactccagggatccatgtttctttcaatagtcagattaagcattccccaatccaatccccagatatctttgaacaaaatcaataaaaatcagtaaaaacaggaatatatatatatatatatatatatatatatatagacacacacacacacacacacacacatgcatatacacacacatgcatggaggaccatactaaggcctttttcaggtcaaaaagggttttcacattgaccttttttacttttaagtatttttcctcagaatgttccttcagttaaaaatcaggtttaatctggagctcttactgatttttctttgattcctactgaacacctagctactggccatggtttctttgaggaaaaaaacaccattgctgaagcatttctaaacatttttaatgcatgcagaaagaactacatagactctccaagcagctatataaggtggctcaagtaacattatgatttattttggtctaagccctttcataacgtccttttaaaatacaaagagaatggctacgaaatggtgccagaacccagaaggcccagctggactgacaggagctctgagcagttcataggacaagcagggacccgccgaacctctcccgtttctgtgctttctctaaatgcagcaggtcctctctttactgcccatgcttttaaactatgaaaaaaaattttttaaagaaatctagcagtgattaatggagacctcaaataacactgtacatgggctttgttagagacaggtaatcattcttaacagctcttttcccagaggaggcctgggtgggccgagaggcatccagagtttaggaagtgcttttattgcagactgcaccttggctaatactatcctctatgtactggctgcctgtgtcactcctgctgaggactgtggaggggatgcgagagggacgcctctctgggttctcctgagagaagcagcagatcatcttcttcatggtgccatacatgtcctcgtccttgtaggagtagatgatggggttcacgacggagttgagcagcgccagcagcaggaaccaccttttcacatgctgcacgccacactgcctgcagttcaggccgtcgaggagcagaaccaccaggcccggggtccagcataccacaaacgcccctaagacagtcatcaccgtcttcattagcttcatgggtgtcctccggcggctgatggacccacttgtatgcggagacaagacgttggttttcctcttgacgtacacgtagatccgcaggtacaccacaaccatgatgaggaaggccatgaggttggacactgtccagaaaacaaggtaactcctgctgtaaatgggggccagggaagagcaggcagagatgttgcagaggcaattccagcccagtgtggggaccgcccccataaaaatggcgatggcccagacaagcaaaatgagcagtgtcaccctctttttggtcaggttgctatggacccgcatcctcatgattgacatgtgcctctccacggcgataaccagcaagttggtgagggaagcagtcaagctactgtccagaagcccctgacggagaaaccagcggttgacagtcaaagtttttgaaactgggcctgtgttaaacatcaggaatacataggcaattccagcgaagaaatcggcagcagctaaattagccaacaggtagtagaaggggaaatgaaattttctgtttttgatcactgccgcgatgaccagagaattagaaaaaaaaataaacaggcagaaaaacgtcccaacacacaaaacaatcacaagctttgttcctgtccagtcatcgacagtatcagtgttgctcctattataaaaaaagtccatgtgcttgtcatagtgacactcattcattgtggagaagtgaacatcctgtaagttggaacataaacaggcctgtgatccactttgaacacccagcagggaaaagcctttgggcagcctaaatcca

SEQ ID NO: 15866 - RNA, 3547 nt, Homo sapiens
  source 1..3547: mol_type = other RNA
gctgggattacaggcatgagccagtgcgcccggcccaggatattcttattcagtgcttctcaatttggttaagcattagaatctcccagagagctttgtaaaaatacccatgcatgggcctcattgtccaacattctgactaacttggtctagaaaggggccctggcaacaatgttttaaaaactccttacatgatgattcaatgtacagtcagagctttaaaaagtctcaatatccaggctgtaccttagatcagataaatcagaattttgcagtgtgaaacccagacatcagtacttttttaaaaacatgccctggtggctgggcacagtggctcacatcttgtaatagatctttgggaggctgagatgggcagatcacttgaggtcaggagttcgagaccagcctagccaacgtggcgaaaccctgtctctactgaaaatacaaaaattagccgggcgtgatggtgcacgcctgtgatcccagctacttgggaggctgaggcatgagaatcacgtgaacccaggaggcggagctgagatcatgccactgtgctggagtccagcctgggccacagtgtgagactctgtctcaaaaaacaaacacataaacaaaaaaagcaaacatgccctggtgcttccaatgtatacccaaagtttaacccaattgttgcaaccccctgatctaactggcttaaaggttaagggtgtgattgttttttcttctgtcctgaagtaagtcagttctagatcatcaccatagtagggccaccaataaagaattctaagcattatccactctggtggtggtgtattcataaatccttccccagtttctttaaaaaagcaaaaggggcaggaggaagaaggtacagaaatcacatgagaaacatttaaaaatacttttagtaaaatactctgtaccctgtcaaaactcctttggcacacagtaaatcatagtgaagaacaaacatagcagaattgccttagttgaggctacagtgtaagagagaatacaacttagaaggtaataatagaaaaatcatagcattttccagcaattgatatgacagtaaatttataaagaaatacaataatttcccagtgactcttaactgttcaggatgccagtgctaaaccaggttgccatacataattcaaagaaagctagaaaacacattccacatattaaattgaagataatttttgttcagagagcaactgaaacatatagtaagttatatattttttagatataagataaaattcttttgcttttagttaaaatgatttttttcatacattctaatggacatatgaaaaagatatttactttttttcatcactaaccctgaggaaggaagaacaaatgtggagtaggccacaaaactcactaggaaccaatctccacacttttcccaattgtgaatagcaattaatgggagaagttcaggatactacacttgtttaggctcccatacacatcagcttaaactatttaaaatagatacaacatttgggcaactagcacagtggcatttctctgcttcaactgagaactattttaaatatcatcacttttatttcctacactggtttaaacaaacaaaacaaaataagacaaaacttgacattgattatgtaagaactttcagttcaatatatagtaatatgtagggacaatatagcttcattgctcaagacttccattcagcaggaaaaaaatgcataagttctaggaattcttctctttcactagaaagacgctagctattacaggggagttgatgagaggaaaatgtgaaatcccatctcaatggaatacaggaggaactggcatttccgctttgccattacagttattattcttaggatgaaagttggaattgcaaatttagctggactcaccagtttcaacctgtggaaatgaaataaagttcaccccctgggccaaaaaccccaagcagcagttgggagcaagagggcaataagaacagaagaaaacagattcactgcgttgttatcaagaatgggtttccctgctatgtgccttgccttatttgttgggctgttgaccaccatgccagtgctttcatccaacccagtatactgcattgtagcccctaagtatgagtccacaattgatcctagtaatccagctaaaccaccaaatgcaataattggccactgcggggcagaaatgtctaaatcattcacaaaaatcagctgtgtgaggaagtatgcaatgcccacaaaggtaccaccaaggagactggagacaaggcccaccactgtaactcctccattggtaccaactggaactttctcccaggttgttatcagtcttggagaacttttactcagaactgggccaacttctgaagcccatgtgtctccagcagagcaggccagtgcagccaagagagacaaacacatccaggaagcggagtactgcttggaaaaatcgactgggatttccccggggccattttctatcatgtacagcagggccagttctgtgggtacagctccattacagaacacctgaacccaattcctttgcccaccttccttatattctgaatctagacgcttcttcacttctcccttccatttagtgagtttcgaagaagacaagaaaaacatcagcaaagaggtaaaaaagctgaaatttgcaatggttaggataaatccaacgactagccctcctagagccccactgtgatctagacttttctttttaaggccattagagacgatcagaacaggaacaacaacagaaaacagccaacgccacggagaaataggtcgtaagttaccataataggtgcttgcagtcattgatataatccagaaagctaacgaaatgcaaatgatcaggctcagtataactatattagttatcatctttatatatcttttgcatatattgtcgttaagatctgtcatggaaaataaggatatgagctcctgcgggaaagaatatttagcgtttcggagagaaagtcatttacgatgtgagcaagacacttgttcagaggcaaacataaatcccaacatattccaccgaccaaacaagcataaaaatcacaaaaattcaaactccttccggaaactcctactggcggagagctccaattcatatgggcgtggtcaacgcctcaccgcaaaagcagagcgcaacccggcggacggtgagggccggtcgccggctgccggccgcttcagcgcctcacgccggagcccacggggaaaagagaaagccgaggcagccaatccgcggtcccggcgctggcgagttccacccacctcccgtcgcaaccttctcacccgcgggccgggtaggccagcggctgcaaaggggcagctagggcacccgaacttgggcaagtctgggaagcacgcccgacgcggctgaacgcagtcacgtcccgacagctgcgcaagccgccctagggtcaggtccagccggccaaggccgagaccccaggagcaaagcccgcgcctcccggcgcccccgcctctagcgcctcgcccgctgtgggcat

SEQ ID NO: 15867 - RNA, 2188 nt, Homo sapiens
  source 1..2188: mol_type = other RNA
gctgggattacaggcatgagccagtgcgcctggcctagatttttctaaaaacaaacaagcaaacttagattttagttttatttgataaaatgagacgttgtacagaatctgtccttatatgagtaaacttatatatgctaagcactagatcgaaagccccagcaacttctcaggtggcagtcacgttgttgcgagggtaacctgaaaacagctgtcagctgggagtaggagccagggtttttttctcagtattcaccttcgggggcacaagtgaaattcagtccgtagaactcattgactacaagaatctcactgcaatatttttggaatgtaaaataactgatgattttaaaaggaatgggcatttcttgtatgtttctgaggaatccagatccaacaagcacccccgcaatggacagcagagccactacactgttgactatatttggattttggacgataccaagtagcacaagagttagaaattcaccaattaagtggggggccaagagagcagcagaaaaatatccaaatcgggcaacctcaggatgtaagcccagcgtccagtagcacacactgctgaaaatcatggtggcaacaacgctgaaggggaggacgtgcagtgcataggccagcatcatctgccacttctggtagaggccgtcctgactctcctggtcgctgacagctcgcagcacgggaaacagattcacagcgttcagcatgcctgtgtacggggtggcgcccacaaactggtaaaggagacctacgcggtcctggatagcaccctttagcacattgcttcggacccgcagaacgaagaaaaggaggaacaaacccatgatcagattctgaaggagacgcgtaatcactgccagcttatttctcaccaagtttcttgtcactctcctcaggagaacacccagtttagagaaaactccaggagaatctttggttttgaaaggaaccattggtaacgttttcaggtgtttcattctttcaatattcttcaaagttttatgacaaattgctgatttcttgtaggcagattctatcatctggactctcttggaggtttctatttcccgttccttgctttgggtatccactgacgtcaggtccatatagaagtcaaaagggtttgaatgttcaggacaagggtaaccgcagtcattgaagaaatcaagcatttccgctggcgtgccacagaaaatcagctctccgaagctcaggatggcaattttgtcaaagagctgaaaaagctcagaacggggctggtgaatggtgagaaccacaattcggttcctgcgagccagttccaccaggaggacgacaatctgattagcagtcatgcagtccaggcctgtggttggctcatcaaacagcatgaccttaggatcctggagcagctgggctgcgatggagacccggcgccgctcacccgtggaaatgccccccaagctgtagttgccaatcagtcggtctgccacatggctcagactcagctctgccatgacggcctccaccttcttctggaaggagccgggattgccgcggcggatggccagcagcgcggtgtagtgcagcgtctcgcgcacggtgaggctgctcagcagggtgtcgctctgcaggacgtaggagaagcagtcctggaactgctcccggcgcagcgcccggccgttcacatacacctcccccaggaaggtccccgcgcgccccagcctcccggacatggcgtccagcagcgtggttttcccggagcctgagcttcctaggatgcacatgatctgcccgctctccacgtacaaggagacatctttgaggatctgcctggtccactgctgccggcaagatgtgatgtcccaccagggcctcacgcggtggctgacgctgtaggaggcatggaggatgcccaggctgtgaggctccggggcggtggcaggagccccctccagggagctctgggagcctctgtttacttggagacccatggaccctccgggggtcaaagatgagaggtcacccatggccaacaggcagcaaagctgggcaaattttctggtggccggaccctccccagagtggcttcagttggggagcccgtggcagactgccctgcctgctccacctgaccccggagtcccttgggacagcaggactgggacttggccacggagaccattatctg

SEQ ID NO: 15868 - RNA, 15320 nt, Homo sapiens
  source 1..15320: mol_type = other RNA
gctgggattacaggcatgagccatagcacccggccctttacatagattttttaaagtagtttcaggtattatcattcatacttgatttataaactctttgacagaagggaccatgtatcttgtatcttgcacttcttttgattcatttacttaacagctacttattgaatgccaactctgtgcccaagtatcaatgtattaacagctacccaattttgtaaaaagggtattggggctggaaaatatgaagaacagctccccagaagattccatgtgacagcctatgagcaaggagatcaggacagatagaaaaaggtatttacaccccctgcgatattgggagtaatatcatcctctcccccctggatatttaatccttataaccgcctctgagatgtgtgctaaagaattcacacttggctgggtgcagtggcttatgcctgtaatctcagcactttgagaggccgaggcgggcagatcacctgaggtcaggagtttgagaccagcctggccaacatggtgaaaccccatctctattaaaatacaaaaattagctgggcatggtggtgcatgcctgtagtcccagctactcaggaggctgaggcaggagaattgcttgaacctggaggtggaggttgcagtgagtcaagatcgcgccactgcactccagcctggcgacagagtgagacttcgtctcaggaaaaaagaaaaaaaaagagaaagtattcacactttacaggtgattaaatcaaaagcaaacaggcccaagtaatctgtccaagcccaagaagctagtaaatggaggagtgagaattcgaaccctggcattcagaacccagagccagagctctttgccacattgtcatactgccttcctccttattacagaggtgcatatagtagccatttcattaaaaatgtaataaatgaatgttcattgcagggctctgatagctcctcattccttccaaagtagcaaaccaggcataaataaaagatgagatacataacttagaaacgtttacataaatttctacatattagaaatttagcacacaaaatggtacacattatgcaagaatacaaacaaaaagatgttaaacatttgagaatggttatgtatggagcattgtaaataaacaggaatagacaaaacaagagaggcctcccgatatcgcatggacatataatgataatgtgccatgaactgaaaatacaattatttggcactcagcacctgaggtcttagcacctgggcccacgtctccagaggtgaagagcagagtcacatgcctccctcctcccccacggaggtctcccaccattctaacctcacagggcttggggtgggatgagatttaaatttatatgaaaatacttacaaatattttaaaattatttcttactgttgctatatttattatataaaaatatgaatacttaatcatttttaggtgaggctagtgtaaaaaaatggaccttccaatcaaaactctataaataaaaattttaaatgttatcttggttctcatccttggcaatgattcttaaatatatctctatatattaggaatctgcagctctgcagtgtggcccaggcatctggtagtgtgtgtatgtacgtgtgtgtgtgtgtgtgtgtgtatgtgtctgtgtttatttctgtcattgctttttttaaattttaacacattttcagcactccaaaaaagaaaccaatacactttaagagtcactcctcattctccagtctcacacctgacccacagtcccaggcaatctcctttatgtctctttagagtgactcaatttccggacattttaacctactttctgtatcttggaattggtctattctggacacttcatatagatagaacaatacaatatgtaaccttttgtgattggtttctttcacttgacataatattttgaagtttcaaccatgttgtagcatatgtcagtatttcattccttttttttaaaaatatactttaagttctgggatacatgtgcagaatgtgcaggtttgttacataggtatacacgtgccatggtggtttgctgcacccatcaacctgtcatctacattagatatttctcctaatgctatccctcccctacccccctacccccagacaggccccggggtgtgatgttcccctccctgtgtccatgtgttctcattgctcaactcccacttataagtgagaacatgcggtgtttggttttctgttcctgtgttagtttgctgagaatgatggtttctggcttcatccatatccctgcaaaggacatgaactcatccttttttatggctgcatagtattccatggtgtacatgtgccacattttctttatccagtccatcattgatgggtatttgggttggttccaagtctttgctattgtgaacagtgctgcaataaacacacgtgtacatgtgtctttatactagaatgatttacactcctttgggtatatgcccagtaatgggattgctgggtcaaatggtatttctgtttctagatccttgagaaattgccacactgtcttccacaatggttgaactaatttacactcccaccaacactgtaaaagcattcctatttctccatatcctctccagcatctgttgtttcctgactttttaatggtcaccactctaactggtgtgtgatggtatttcattgtggttttaatttgcatttctctaatgatcactgatgatgagcattttttcgtatgttttttggccacataaatgtcttcttttgagaagtgtctgttcgtatttttcacccacttttggatagggttttttttttcttgtaaatttgtttaagttcctgtagattctggatattagccatttgtcagatggataggttgcaaaatttttctcccattctgtaggttgcctattcattctgataatagtttttttgctgtgcagaagctctttagtttaattaaatctcatttgtcaattttggcttttgttgccattgcttttggtgttttagacatgaagtctttgcccatgcctatggcctgaatggtaatgcctaggttttcttctagggtctttatggttttaggtcttacatttaagtctttaatccatcttcagctaacttttgtataaggtgtaaggatggggtccagtttcagttttctgcatatggctagccagttttcccagcaccatttattaaatagggaatcctttccccatttcttgtttttgtcaggtttgtcagagatctgatggttgtagataagtggcattatttctaaggcctcacttctgttccattggtctatatatctgttttggtaccagtaccatgctgtttgggttctgtagtcttatagcatagtttgaagtcaggtagcatgatgcctccagctttgtttttttttccttaggattgtctcggctatatgggctcttttttggttgcaatatgaactttaaagtagttttttccaattctgtgaagaaagtcaatgatagcttgatgaggatagcattgaatctacaaattactttgggcagtatgaccattttcacaaaaatgattcttcctatccatgagcatggaatgtttttccatttgtttgtgtcctctcttatttccttgagcagtggtttgtagttctccttgaagacgtccttcacatcccttgtaagttggatttcttgttattttattctctgtagcaattgtgaactggagttcactcatgatttggctgtttgtctgttattggtgtataggaatgcttgtgatttttgcacactgatttttatatcttgagtttgctgaagttgcttatcagcttaaggagacttggggctgagacgatcgggttttctaaatatactatcttgttatctgcaaatctgcaaacagagacagtttgacttcctctcttcctatttgaatacgctttatttctttctcttgcctgattgccctggccagaacttccaacagtatgttcaacaggagtggtgagacaaccttgtcttgtgccggttttcaaagggaatgcttccaggttttgccctttcagtatgatattggctgtgggtttgtcataaatagctcttattattttgagatacattccatcaatacctagtttactgagagtttttagcatgaaggtgtgttgaattttatcgaagaccttttctgcatctattgagataatcatgtggtttttgttgttggttctgtttatgtgttgaattatatttattgatttgtgtatgttgaactagccttgcatcctagtaatgaagccaacttgatcgtggtgggtaagttttttgatgtgctgctggattcagtttgccagtatttaattgaggattttcacatcaatgttcttcagggatattggcctgaaattctctttttttgttgtgtctctgccaggttgtggtatcaggatcatgctggcctcataaaatgaatcagggaggagtccctctttttctattgtttggaatagtttcagaaggaatggtactggctcctctttttatctctggtagagtttggctgtgaatctgtctggtcctgggctttttttgttggtaggctattagttactgcctcaatttcataacttgttattggtctattcagagatttgacttcttcatggtttagtctggagagggtgtatatgtccagtaatttatccatttcctctagattttctagtttatttgcataaaggtgtttatagtattctctgatggtagtttgtatttctgtgggatcagtggtgagatcccctttattatttttattgtgtctatttgattcttctctcttttcttctttattagtctggctagtggtctattttgttaatcttttcaaaaaatcagctcctggattcactgattttttaaggatttttcatgtctctatcttcttcagtgctgctctgatcttagttatttttggtcttctgctagcttttgaatttgtttgctctttgcaaaagaacaaaatttgttcttttaattgttatgctagggtgtcgattttagatctttctcactttctcctatgggcttttggtgctataaatttccctcaaaacactgctttacctgtgtcccagagattctggtacgttgtgtctttgttcttattggtatcaaagaacttatttatttccaccttaatttcgttatttatccagtagtcattcaggagcagattgttcagtttccatgtaattgtgtggttttgagtgagtttcttaatcctgagttctaatttgattgcactgtggtctgagagactgttacgatttccatgattttgtacttgctgaggcattttttacttccaattatgtggtcaatttcagcataagtgcaatgtggtactgagaagaatgtatattctgttgatttggggtggagagttttgtagagaacttgctttgtgaatctgggtgctcctgtattgggtgcatatatatttagtatagttagctcttcttgttgcattgatccctttaccattatgtaatgcccttctttatcttttttgatctttgttggtttaaagtctgttttatcagagactaggatggcaatccctgcctttttcccttccatttgcttggtaaatattcctccatccctttattttcagcccatgtgtgtccttgcatgtgagatgggtctcctgaatacagcacactgatgagtcttgactcgttatccaattttccagtctgtgtcttttaattggggcatttagtccatttacatttaaggttaacactgttatgtgtgaatttgatcctgtcattatgatgctagctggttatactgcccattagttgatgcagtttcttcatagtgtcagtggtccttacaatttggtatgtttttgcagtggctggtaccggtttttcctttccatgtttactgtttccttcaggagctcttgtaaggcaggccttgtggtgataaaatctctcagcatttgcttgtttgtaaagtatttcatttctccttcacttatgaagcttagtttggctggatatgcagttctgggttgaaaattgttttctttaagaatgtcgaatattggcccccactctcttctggcttgtagggtttctgcagagagatctgctgttagtctgatgggcttccctttgtgggtaacccaacctttctctctggctgcccttaacattttttccttcacttcaaccttgatgaatctgaggattatgtgtcttggggttgctcttctcaaggagtatctttgtggtatcctctgtatttcctgaacttgaacgttggcctgtcttgctaggttggggaagttctcctggataatatcctgaagagtgttttccaacttggttccattctccccatcactttcaggtacaccaatcaaatgtaggtttggtcttttcacatagtcccatatttcttggatgcttcattcattccttttcattttttttctttctaattttgtcttcatgctttatttcattaagttgatcttcaatctctgatacctttcttctgtttgattgattcagctattcatacttgtttatgcttcacgaagttctcatgctgtgtttttcagctccatcaggtcatttatattcttctccaaactggttattctagttagcaattcttctaacattttttcaaggttcttagcttccttgcattgggttagaacatgcccctttagctcagaggagtttcttattacccaccttctgaagtctccttctgtcaattcgtcaaactcattctccatccagtttacttcccttgctggcaaggagttgtgatcctttagagaagaagaggcattctggtttttggaatattcagctttttaccctggtttttcctcatcttcatggatttatctactgttggtctttgatgctagtgaccttcagatggggtttttgtgtgcaagttcttgttgatgttgatgctattcctttctgttagttttccttctaatagtcgggcccctctgctgcaggtctgctagagtttgctggaggtcccctccagacacagtttgcctgggtatcatcagtggaggctgcagaacagcaaatattgctgcctgttccttcctctggaagcttcatcccagaggggcacccgccagatgtcagctggagctctcttgtatgaggtgtctgtcgactcctgcagggagatgtctcccagttgggaggcatgggggtcggagacctacttgaggaggcattctgtccctcagcagagtttgagcactttgctgggggatacgctgttctcttcagagccagcaggcaggaatgtttaagtctgctgaagctgcgcccacagctgcaccttccccaggtgctctgttccagggagatgggagttttatctataagcctttgactggggctgctgcctttctttcaggagccctgcccagaaaggaggaatctagagaggtattctgactacagcagctttgctgagctgcagtgggctccacccagtttgaacttcccagcagttttgtttacactgtgagaggaaaatcacctactcaagcctcagtaatggcagacaccccttcctccaccaagctggagcatcccaggtcaactgtagactgctgtgctggcagtgagaatttcaagccagtgggtcttagcttgctgggctccatgggggtggggtccactgagctagaccacttggctccctggcttcagccctttttccagggaagtgaatggttcggtctcgctggtgttccaggccccactggggtatgaaaaaaactcctgcagctaccttggtgtgtgcccaaagggccgcccagttttgtgcttggaacccagggcccttgtggtgtaggcaggcacctgagggaatctcctggtctgcaggttgcgaagacagtggaaaaagtgtagtatctgcgcctgaatgcactgttccacgtggcatagtcccttatggcttcccttggctaggggagggagttcctggaccccttgcacttcccaggtgaggtgatggcccaccctgcttctgcttaccctccatgggctgcacccactgtctaaccagtctcagtgagatgagctgggtacctcagttggaaatgcagaaatcacctgccaactgcattgatctcgcttggagctgcagatcgcagctgttcctatttggccgtcttgccagccccctcattcgtttttaagactaaatgatatttcattgtatgtagatgctaattttgtttatccatttatctattgataggcacatgctaattttttatgattacgaataatactactatgaacatttatgtgtaagttttgtgtgaatgcatatttttgtttctcttggctacatacctaggaaaataatttctgggtcatgtgggaactctacatttaactttttgatgagtttaagcatcttcatgctttaaagttccctggaaggacaaggacctggctctctgactccccaggctgtctcttgaaaggtccacactccaggtcaggtttttgagaagttactttaatgttttatgaaaagagaggtgtcttcacttcaactttttaatgaaaagattcatcataatgattattatctccctttcatcatacctctctccttagctctatatactttgagaatgacattattcacctttttaagtaaataggtcacatagcacagttatgagcacatgctatagaggcagccttcctggcttacatgctgccttccctacttaccagctatataattttggccatgttacttaacagtttctcatgtataaaaatgatatgatgacaatatgatattactttcttagggttattgtggaaattcaattaattaatatctgtgaagtccatagaatggtacctggcatagtctaagtattctataaatgttcatttttattatcctactaccaacattccacaatgtttgtcatacagatggtgctccacgagtatttgctgaatgagatacatgataagagggcttagctagagcaagactcatcacatgtaaagtattaatagaatgaaccagtccttcccatttgttcctagggaaactaatcactccttcctggttgcacctacagcacttagaacatccaatagagctgacatctgggccttggaatattgtggctgtgctcatatctgtggctcacaaacagctccaaactcttcttcacctttttatagctgacacccagcagaggagccaagcactaagcaggtttgcaaatattcaatgcaacaccttattggtacttgattggcaataagaccagtcttaaataaaatctatatatatatattagccattaaccaagaccaccaagttttatgtgcagttttataattagctagtagtacgacatttgaccatatagctaccctcttttgtgttttcctaaggtataatattggcccagatgaaaatgggatttgtttggttcaaaaatcgtcaaaaatcagctatttcatatgattcaagctgatacttccagccctcaagttctatgccctaagcaagtagttctcaaaagactcctttagtcgagaaagaaaaaatactccttatgacagactcgtacaacataacgtacacacaagcatgagtgtacttaataagcataggtaactttgaagcacagcactaaacgaagggaaatacgtatttattaacagtcaggaccacaatcccatttaaatttcaaacaactttcagaaataggtatctcttcacattacaaatgaaagaaacagatgccaaatgaatcacttgtaaatgatacagaagtattaagtgtggatccaggactcccacctacccccaagtctatctgaatatagagcctatgttttccccaccacgaccctctgctttcgctgaggaagcctaacctacacagaatggccctggaaagaatgactaaaggataagcagccaaaaccagaatggaaaataattcgtatactctaattttactgcaggatgcaactgcaattttatttcagtcgtaccatttattatgaaatatctcttcttgatttcctccccaaacctgacattgaagtctcgatggtaacattaaaaaatctcttagctatatccttaagggttcagaataaaatcttcctgtacatgataagaggcagcataggtcaagagcctactctgatttctgcttcttggtgatcatacaacttcatacaagttacttggcctcctcttgcctcagcttctcacttctggaaaaattaagaaaatatcagtaactatcatggaattttaaaacacaccttccttttcttacagaaaaaaaaaagaggagctaaaaaattatatttctggggttttttgtttgtttgttttttgtccattcttggttaaaaaggaatcagctaaggaaacttgaaggcaaaagagtgacgtagaaactacagatactttattgataaacagttgatgtaaatatcttattttgagtaggtgatgtaatggaaatggtactaaaacttgattaagtaaagacaaaactggccaggcatggtggctcatgcctgtaatctaagccctttgagaggctgaggtaggtagatcatctgagcctgggagttccagaccagcctgggctacatggcagaaccctatctatacaaaaaatacgaaaattagccaggtatggtggtgtgcacctgtggtcccagctacttgggaggctgaagtgggaagattgtgtgagctgagaagtcgaggctgcagtgagctgagattgcgccattgcactccagcatgggtgacagagtgagaccctgtctcaaaaacaacaacaaccaccaccaaacaaacctaatatgttatgaataaatttaactctgtaactcctctgtataagtcatggcagttttcctcttgtgtgatttccttcttttcactataaaaaaaatgaggactcttctgttgtcgaactttgctaaatcatattaataaaatgtatgccagttaaggtgtgattttttctttttctcttctttcttttttctccaaaaagccatcacaagagagaacaattttgtttttttttgagataacgactaagattaatgtggtcccttttatataagctaataagacaaattgtttttaatttttaaacaaaattattattttttagagacacggtctcactctgtcacccaggctggagtgcaatgacagtattactgctcactgcagccttgacttcccaggctcaagggatcctcctgcctcagcctcctgagtagctaggactacaggtgcacaacaccacacctggctaattttttattttttgtagagacagggtctcatcatgttgcccaggctggtctggaactcctgggctcaagtgatctgcccacctcagcctcccaaagtgctgggattacaggtgtgggccactgtgcccggcctataatattttaaattgtaaaattaaaacattaataagtttctaaacctgaatctaacatgtggctttatgtcctgataactccacatgatgttacgatgattaaaggagtaaattcatgaaaaacacttaggacagtgtctggcacaagctaagtgttcaggaaattattattattagtgttgcatcttaatggtctcaagctattatttttcacccatcatatttagtgtaaaatagaatttggccctgggaatcaatgaccacatacatggtataactaatctcaaatatttaaattgactaagatatctatgtttcattaaggtaatcttggcccatagagtctaactagatcaatcgtttacaatcattaaaagaaaaaaaagtgaagcacataatgcaaaaacatttcacaggactccatgtgatataaattatataaattgttattttgttttatcccctagctgaaaaaaatacataaagagtaaaagctaccataaatcctctaatgctttgaaattaatttgtattttgtttttgacaacgtatatttgaaaatttatatttgagccatattcattcacacggcagttaagcttgtagaatatacagattcactggcgttttaatagcttaatgagctcctgggaagccatggctagccattaggaataatgagttagaaaggtcagcaaaaccttttctgcaaagggccagagagtaaatatattaggctctgctggccatgtatgtctctgttgaaacaactcaactttgccattgtagcagtgggcaacatgtaaacaaatgggtgtagctgtgttccaataagacttcactttcaaaagcctcagcccacactgaaggtggggaggttatgcaaaggtgtaaatgccaggcagcaggcatcactgggagtcctcgcagaggctgctggccacataacccaatgctcacgatccccaaagtgtatttggaggaacatgaattgttgatgtgtttgggaatttttttgaagctgcattttatatttaaactatattttcaaaatttcacacaggagcttcaatcaagctgtgtaataagtatatgggagtcatttatattattctctataatttatttgtaatatatcaaaacaaaaatgcctcaaaaatatacagtaaaagaatcaaacacattcctagagttgtttttatgaacaatctgtttatatagtgctggtttatgttttatatcttgtcataattttaacatatgtttaagtatgaatgtttatataatagtaagtttctctcatagaccatctctcttctgcttaccacatttcctttaacaccctaattacaacgactctgagattctacctgaaaaattagcaagatgcccccacattctagcttttctctccacaaatattgaggaaagtcccagctttgtttacacatgtccttgagtcagacctcattgccacctactgatgtgatataatttgggtgtgtgtctcctccaaatctcatgttcaaatgtgacctccaatgttgcagatgagcctagtgagaggtgtttgggtcacgggggcaaatctttcatcaatggcttggtgccatcccaatggtaatgagtgagctctcattctggcagttcacacgagagctaggttatttaaaggagactgggacctcctcctccctctcttactacctctctcctgccatgtgatatgtccacttcccctttgtcttccactatgaatggaagcttcctgaggccctcccgaagcagatgctgttatcatgcttcttacacagaactatgagccaaataaacctcttttctttataaattacccagcctcaggcattcctttatagcaatgcaaggtagactaacacgtgatgctcatttttttttaaagcctgcaaacagtaagaagattcccctctctttctcagtggatgtaaagcagtgattctgcataaatgtatcaacactatagctcaactccttctggagtggacttcccctagacctggagagcgagtcctgcctagcatacacggcctgaagttcgagatctcttccaattcaggtaatattccgctttctgtatgcctgatctctacatatatctgacattgatttttaactcaaatgaggaaacaggaaattattaattacaatctcctaaaactacaacaggtgttataaaacttctgaatataaacaggcagacagcaaaaatgtacacaggcataaaatgtaaacttgagtgagaaaaaggagctgaaaaatgaaaggctcgctttgaaacaaaacagcactgaagagtctacaaagagagagtgactggagagagactgatgtgggagagcagaatggggatcagattataatgagtatctctcccacactaaggaatttgcagctttttttgataggcaataaagagttacatataacagctgtatttaaattgttcctaggtgatggagctgcaggtaattcttttcttcttcctttttgtattttactttttctttttttttttttttttttgagacagagtctcactctgtcacccaggctggagtgcagtggcgtgatctcagctcactgcaacctccacctcctgggttcaagcaattctcctgcctcagcctcctgagtagctgggattataggcgcacaccaccatgtccagctaatttttgtattttagtagagacggggtttcaccattttggccaggctggtctcgaactcctgaccttgtgatccacccaccttgatctcccaaagtgctgggattacaggtgtgagccactgcacctggccttaatttttgtttattggaaaagaaggaaaatctatatttttaaggccaccagccacagcacttagagaagaaggaggacgtatattgcttttgctgtttcctgttagcctgacatttgcgactacattgactctgctggggtcactttctctaatttgtggatttttttttctttctcaactgcctggaggatatgtatgggtccatgactcggccaccacataagattgtgaagattatacctgtcaagggtgcccagtcaaggaagaagagtggctgaattcagcctgtgctctgcctgaaagccctatgctctgtgtgggccttagtccacctagaggaaggggtaccttttaaaagtacacacaaaggcacatcatgggctggccgcagccctgcctggccccaggtgagctagcagtgccagatgcctccagaatagactggaaggccttctgtccctctattatgtcaaaactgcaactggaactactttgtccaaggaaaggagagagaaaccataggaaaaggccataggagaatggtgtctggaaaaaaaaactgcaacgaatataagagatatgaatgaagcagatgcaatgaaacaacaggtttaatttcaggcttattttagcgaatggaatagaatccccattgagtaaacacgaatacaaagggtttattgagaagatacagaggaattgcacagagccaaaagcccagtctggcttcacaagacttggaaaactagagtgaggttcaaggaggttttccccgttcatttctccagagtcacacagcctctcctctcctcacctctgtactgtctgctctactcttcagtctctctctaaagacaagtttttcttactcgttagaaagctcacggcaaaaaatggctcctcgat

SEQ ID NO: 15869 - RNA, 918 nt, Homo sapiens
  source 1..918: mol_type = other RNA
gctgggattacaggcatgagccatatgagtgaagcaggggggtgagatcaaggctgggagagacttggaatggcagttctgagacaaggatctgggcgcaggaggtttatgtgtcaggtgattccgaggcacaagggaggggagggggaagggggacaggagacggggagccaacagtggctgcattaaaagcctgttgctagtgtgggcgcctggactccattctgttagaatcatctgaggacataagccaaactcttattggtgaggtttgctgtggacagcattaaaccctcatcagttctgggctgttctacagatagtgggagtgatggcacgtctttgtacccatcactggtgggttgcagggtggggaaaggctggtggcaggggccctgattaggggagagcctgaataagcccttcagctgaacttagaggggtaaggagccttcagagaggctggaggctgtgcacatgtcaccagtgagtgcccgtgagcctggaagtggctgctgcttgctggacacactggagtctggcagggtcagctgagcagctcttgtctcctcggctgtccagccagcctggcagcctcctgggacctttgatgacttgatcctagtgcccgcctgcctccacggctgctgcgactcagtttccttggctgtccctcctctcggtgaccttcagcgttgaggagtcttcaaggtctagctctggacagttgtctctgctctctgaactctcacttcctggcctaaaatgcaggcagagttggtgttggggaaggagatggctgtgggtccattatactccatgaagccagaggagcctcacagcagcctcctgggaacggaaggttaccaggcaatccggggctgggtcacttctctgccggcctgtgctagtctccct

SEQ ID NO: 15870 - RNA, 2466 nt, Homo sapiens
  source 1..2466: mol_type = other RNA
gctgggattacaggcatgagccatatttttgtattcttagtggagatggcgtttcaccacgttggccaggctggtctcgaactccggacctcaggtgatctgcctgccttggcctcccaaagtgctgggattataggcatgagccactgagcccagccccaattttgctttcaaggggcctttgcccaccctcagtgggtggctgccccacagaaggtacttaattagggactattgttgagacagaaagaggaggtgggcatctccttcccactcccccagagctgactggactagaggcaaggcctttgcagacagacacgtctgtcttgggaagcaagctcttgtcctagcttttggtctgttcatgttttatcttctttggtcaccattagggacaggttgccagatgagtcagagaaggttccatcaagccccttcccctgagaaaggtcacaaagaccttgtgccggagggtggagagaggatggcaacatcttagctcaaaagtctgccccaaggtagtgccatacagtgagggcagtgtcctttcctaacccagtctacctctatcacttgagagtagttgcccaaagctttttttttttttttttttttttttttgagatggaatctcgctctgttgccaggctagagtgcaatggtgcaatctaggttcactgcaacctctgcctcccaggttcaagcgattctcctgcctcagcctcctgagtagctgggactacaggcgtgtgccaccatgcccggctaatttttgtatgttttagtagagatggggttttacaatgttggccaggatggtctcgatctcttgacccatgatctgcccacctcggcctcccaaagtgctgggattacaggtgtgagccactgcgcccactcccccaaagctttagaccgatgccccatcggggagaactaggtggtttaaagtcttcccccaaggtctgcacctggccctgacattccttccggccccataagattaagggactcaggataaagtcatcagtcacagttactgtagtatgcgcccacaggcggatgaaggggctcatttgagttctggattttccaacagcctggctctgccatcatccctgcccaggtgaggtagcctccaaatctaatggcccaccagtgcccacagaggtggtgcccagaccacagtagatatcccttcttcccccagctcagtccatgatgttcatggaggagaagacttcaggcctggaagcagggactaatttttgagggaattgccagggatctggttgaatggcacaaccacttcagtgaccgtatccgtggtggcccgggagcatttccggctactgcgcatgctgtagaacttttcggtgaggtgcttgcggaacttcttggtgaggaaacagtagataacagggtctaagacacagttggtgctaaggaggcagagggtgacctgatgtgcatcattaatggcctggtggaatttgctgtcctggaagcccagctcagcaagggtccagggcagctgcaccacgtggtggggcacgaagcagatgatgaacaccgccaagaccgtgcacaccatccacagcgcccggcgcttgacttcagcgttgcgctgctgctgcaccggctgcatgagcaaggtacggatgatgaccaggttgcagaagaggatgatgaggaagaccaggaagaagctgaacacgatgaagatgtggatgatgaggactggcacgctgcccttctcgtaatgctcaaagcagcgagtgacgttgcctgagccagcactgtcgggcactgtgttggtggagtccaggatgaggaagtaggatgcagctcccacaatggccacccagatgaccaaggacaaagagatgccacgcttgcgggtgttggcctgagcagtcttgatgggccgagttactgcctggaagcggttataagtgatgacgcccaggaaggccacagagcagtaggtgttgatgaagaaaaggcagccagccacgttgcacaggaatttggggagtatccagttgccctggttttggtagtagacaatccaaagtggcagggtgatcaagaagagcatgtccgccatggtgaggttcaccatgaagatctttatctcattgaatttcttgcaagggtacaggcgggcaaagacccacagcacgtagccattagcaatgaccccgagcacaaagatgatgctgtaaacaatcgggaagagagtgtatcggaactcagagtccatgtgggaggagtcatgtggctccattgctgtgggctggaatgatcagctggtcctggtggtgcctgagaaacagcagggacaatggtccaggcagtgacaaagaggctgaggcagatgggggtcccctgagagcatgtttcctggacggcttctcggggaggtcctggatgacttctcggggagctcaggaagcaggt

SEQ ID NO: 15871 - RNA, 2501 nt, Homo sapiens
  source 1..2501: mol_type = other RNA
gctgggattacaggcatgagccatatttttgtattcttagtggagatggcgtttcaccacgttggccaggctggtctcgaactccggacctcaggtgatctgcctgccttggcctcccaaagtgctgggattataggcatgagccactgagcccagccccaattttgctttcaaggggcctttgcccaccctcagtgggtggctgccccacagaaggtacttaattagggactattgttgagacagaaagaggaggtgggcatctccttcccactcccccagagctgactggactagaggcaaggcctttgcagacagacacgtctgtcttgggaagcaagctcttgtcctagcttttggtctgttcatgttttatcttctttggtcaccattagggacaggttgccagatgagtcagagaaggttccatcaagccccttcccctgagaaaggtcacaaagaccttgtgccggagggtggagagaggatggcaacatcttagctcaaaagtctgccccaaggtagtgccatacagtgagggcagtgtcctttcctaacccagtctacctctatcacttgagagtagttgcccaaagctttttttttttttttttttttttttttgagatggaatctcgctctgttgccaggctagagtgcaatggtgcaatctaggttcactgcaacctctgcctcccaggttcaagcgattctcctgcctcagcctcctgagtagctgggactacaggcgtgtgccaccatgcccggctaatttttgtatgttttagtagagatggggttttacaatgttggccaggatggtctcgatctcttgacccatgatctgcccacctcggcctcccaaagtgctgggattacaggtgtgagccactgcgcccactcccccaaagctttagaccgatgccccatcggggagaactaggtggtttaaagtcttcccccaaggtctgcacctggccctgacattccttccggccccataagattaagggactcaggataaagtcatcagtcacagttactgtagtatgcgcccacaggcggatgaaggggctcatttgagttctggattttccaacagcctggctctgccatcatccctgcccaggtgaggtagcctccaaatctaatggcccaccagtgcccacagaggtggtgcccagaccacagtagatatcccttcttcccccagctcagtccatgatgttcatggaggagaagacttcaggcctggaagcagggactaatttttgagggaattgccagggatctggttgaatggcacaaccacttcagtgaccgtatccgtggtggcccgggagcatttccggctactgcgcatgctgtagaacttttcggtgaggtgcttgcggaacttcttggtgaggaaacagtagataacagggtctaagacacagttggtgctaaggaggcagagggtgacctgatgtgcatcattaatggcctggtggaatttgctgtcctggaagcccagctcagcaagggtccagggcagctgcaccacgtggtggggcacgaagcagatgatgaacaccgccaagaccgtgcacaccatccacagcgcccggcgcttgacttcagcgttgcgctgctgctgcaccggctgcatgagcaaggtacggatgatgaccaggttgcagaagaggatgatgaggaagaccaggaagaagctgaacacgatgaagatgtggatgatgaggactggcacgctgcccttctcgtaatgctcaaagcagcgagtgacgttgcctgagccagcactgtcgggcactgtgttggtggagtccaggatgaggaagtaggatgcagctcccacaatggccacccagatgaccaaggacaaagagatgccacgcttgcgggtgttggcctgagcagtcttgatgggccgagttactgcctggaagcggttataagtgatgacgcccaggaaggccacagagcagtaggtgttgatgaagaaaaggcagccagccacgttgcacaggaatttggggagtatccagttgccctggttttggtagtagacaatccaaagtggcagggtgatcaagaagagcatgtccgccatggtgaggttcaccatgaagatctttatctcattgaatttcttgcaagggtacaggcgggcaaagacccacagcacgtagccattagcaatgaccccgagcacaaagatgatgctgtaaacaatcgggaagagagtgtatcggaactcagagtccatgtgggaggagtcatgtggctccattgctgtgggctggaatgatcagctggtcctggtggtgcctgagtctgcacctgggtctgtttcttccttgctgcgtgatccttggctctcccagcctccttttcttcatctgtagcaggggcagcggcttcagctgcagtgaccgtgtgtctctgtctgggtcctggccccagcctcagcctctatgctgtctggcaattgcagaagt

SEQ ID NO: 15872 - RNA, 2548 nt, Homo sapiens
  source 1..2548: mol_type = other RNA
gctgggattacaggcatgagccatatttttgtattcttagtggagatggcgtttcaccacgttggccaggctggtctcgaactccggacctcaggtgatctgcctgccttggcctcccaaagtgctgggattataggcatgagccactgagcccagccccaattttgctttcaaggggcctttgcccaccctcagtgggtggctgccccacagaaggtacttaattagggactattgttgagacagaaagaggaggtgggcatctccttcccactcccccagagctgactggactagaggcaaggcctttgcagacagacacgtctgtcttgggaagcaagctcttgtcctagcttttggtctgttcatgttttatcttctttggtcaccattagggacaggttgccagatgagtcagagaaggttccatcaagccccttcccctgagaaaggtcacaaagaccttgtgccggagggtggagagaggatggcaacatcttagctcaaaagtctgccccaaggtagtgccatacagtgagggcagtgtcctttcctaacccagtctacctctatcacttgagagtagttgcccaaagctttttttttttttttttttttttttttgagatggaatctcgctctgttgccaggctagagtgcaatggtgcaatctaggttcactgcaacctctgcctcccaggttcaagcgattctcctgcctcagcctcctgagtagctgggactacaggcgtgtgccaccatgcccggctaatttttgtatgttttagtagagatggggttttacaatgttggccaggatggtctcgatctcttgacccatgatctgcccacctcggcctcccaaagtgctgggattacaggtgtgagccactgcgcccactcccccaaagctttagaccgatgccccatcggggagaactaggtggtttaaagtcttcccccaaggtctgcacctggccctgacattccttccggccccataagattaagggactcaggataaagtcatcagtcacagttactgtagtatgcgcccacaggcggatgaaggggctcatttgagttctggattttccaacagcctggctctgccatcatccctgcccaggtgaggtagcctccaaatctaatggcccaccagtgcccacagaggtggtgcccagaccacagtagatatcccttcttcccccagctcagtccatgatgttcatggaggagaagacttcaggcctggaagcagggactaatttttgagggaattgccagggatctggttgaatggcacaaccacttcagtgaccgtatccgtggtggcccgggagcatttccggctactgcgcatgctgtagaacttttcggtgaggtgcttgcggaacttcttggtgaggaaacagtagataacagggtctaagacacagttggtgctaaggaggcagagggtgacctgatgtgcatcattaatggcctggtggaatttgctgtcctggaagcccagctcagcaagggtccagggcagctgcaccacgtggtggggcacgaagcagatgatgaacaccgccaagaccgtgcacaccatccacagcgcccggcgcttgacttcagcgttgcgctgctgctgcaccggctgcatgagcaaggtacggatgatgaccaggttgcagaagaggatgatgaggaagaccaggaagaagctgaacacgatgaagatgtggatgatgaggactggcacgctgcccttctcgtaatgctcaaagcagcgagtgacgttgcctgagccagcactgtcgggcactgtgttggtggagtccaggatgaggaagtaggatgcagctcccacaatggccacccagatgaccaaggacaaagagatgccacgcttgcgggtgttggcctgagcagtcttgatgggccgagttactgcctggaagcggttataagtgatgacgcccaggaaggccacagagcagtaggtgttgatgaagaaaaggcagccagccacgttgcacaggaatttggggagtatccagttgccctggttttggtagtagacaatccaaagtggcagggtgatcaagaagagcatgtccgccatggtgaggttcaccatgaagatctttatctcattgaatttcttgcaagggtacaggcgggcaaagacccacagcacgtagccattagcaatgaccccgagcacaaagatgatgctgtaaacaatcgggaagagagtgtatcggaactcagagtccatgtgggaggagtcatgtggctccattgctgtgggctggaatgatcagctggtcctggtggtgcctgtagcaggggcagcggcttcagctgcagtgaccgtgtgtctctgtctgggtcctggccccagcctcagcctctatgctgtctgagaaacagcagggacaatggtccaggcagtgacaaagaggctgaggcagatgggggtcccctgagagcatgtttcctggacggcttctcggggaggtcctggatgacttctcggggagctcaggaagcaggt

SEQ ID NO: 15873 - RNA, 2430 nt, Homo sapiens
  source 1..2430: mol_type = other RNA
gctgggattacaggcatgagccatatttttgtattcttagtggagatggcgtttcaccacgttggccaggctggtctcgaactccggacctcaggtgatctgcctgccttggcctcccaaagtgctgggattataggcatgagccactgagcccagccccaattttgctttcaaggggcctttgcccaccctcagtgggtggctgccccacagaaggtacttaattagggactattgttgagacagaaagaggaggtgggcatctccttcccactcccccagagctgactggactagaggcaaggcctttgcagacagacacgtctgtcttgggaagcaagctcttgtcctagcttttggtctgttcatgttttatcttctttggtcaccattagggacaggttgccagatgagtcagagaaggttccatcaagccccttcccctgagaaaggtcacaaagaccttgtgccggagggtggagagaggatggcaacatcttagctcaaaagtctgccccaaggtagtgccatacagtgagggcagtgtcctttcctaacccagtctacctctatcacttgagagtagttgcccaaagctttttttttttttttttttttttttttgagatggaatctcgctctgttgccaggctagagtgcaatggtgcaatctaggttcactgcaacctctgcctcccaggttcaagcgattctcctgcctcagcctcctgagtagctgggactacaggcgtgtgccaccatgcccggctaatttttgtatgttttagtagagatggggttttacaatgttggccaggatggtctcgatctcttgacccatgatctgcccacctcggcctcccaaagtgctgggattacaggtgtgagccactgcgcccactcccccaaagctttagaccgatgccccatcggggagaactaggtggtttaaagtcttcccccaaggtctgcacctggccctgacattccttccggccccataagattaagggactcaggataaagtcatcagtcacagttactgtagtatgcgcccacaggcggatgaaggggctcatttgagttctggattttccaacagcctggctctgccatcatccctgcccaggtgaggtagcctccaaatctaatggcccaccagtgcccacagaggtggtgcccagaccacagtagatatcccttcttcccccagctcagtccatgatgttcatggaggagaagacttcaggcctggaagcagggactaatttttgagggaattgccagggatctggttgaatggcacaaccacttcagtgaccgtatccgtggtggcccgggagcatttccggctactgcgcatgctgtagaacttttcggtgaggtgcttgcggaacttcttggtgaggaaacagtagataacagggtctaagacacagttggtgctaaggaggcagagggtgacctgatgtgcatcattaatggcctggtggaatttgctgtcctggaagcccagctcagcaagggtccagggcagctgcaccacgtggtggggcacgaagcagatgatgaacaccgccaagaccgtgcacaccatccacagcgcccggcgcttgacttcagcgttgcgctgctgctgcaccggctgcatgagcaaggtacggatgatgaccaggttgcagaagaggatgatgaggaagaccaggaagaagctgaacacgatgaagatgtggatgatgaggactggcacgctgcccttctcgtaatgctcaaagcagcgagtgacgttgcctgagccagcactgtcgggcactgtgttggtggagtccaggatgaggaagtaggatgcagctcccacaatggccacccagatgaccaaggacaaagagatgccacgcttgcgggtgttggcctgagcagtcttgatgggccgagttactgcctggaagcggttataagtgatgacgcccaggaaggccacagagcagtaggtgttgatgaagaaaaggcagccagccacgttgcacaggaatttggggagtatccagttgccctggttttggtagtagacaatccaaagtggcagggtgatcaagaagagcatgtccgccatggtgaggttcaccatgaagatctttatctcattgaatttcttgcaagggtacaggcgggcaaagacccacagcacgtagccattagcaatgaccccgagcacaaagatgatgctgtaaacaatcgggaagagagtgtatcggaactcagagtccatgtgggaggagtcatgtggctccattgctgtgggctggaatgatcagctggtcctggtggtgcctgtagcaggggcagcggcttcagctgcagtgaccgtgtgtctctgtctgggtcctggccccagcctcagcctctatgctgtctggcaattgcagaagt

SEQ ID NO: 15874 - RNA, 3973 nt, Homo sapiens
  source 1..3973: mol_type = other RNA
gctgggattacaggcatgagccatcaagcccggccctaacagttttaaaatgcactgcattttattacataaaagtacaagtagtaaagtaatatactcatttattttaatatacttttaattatttctttgtgtcactataataaagtattgctctgaacatttacgttatacattacttaatagaattttactacaaacagcttctccacttgtattttcattatgcgtcttacattttaatgttcttactattttatagaaaaagtcataatgtccaaataatgtaaaaaaatcgaatatctctgatgcagaagccactgatcacatgctttctcacatgtgaatagaaataaaataacagcataatttgaaagctgtattacatcattattcagctttcaaaaaattttattcaaggaaacaagtatactttcaacgtaattacaatgcttccaaaaatctactccttttaaagttaaatagaaatcatttacctaaaaactgcagttgtggattagtttttatattcaatgctctgatttagtgtaatgtctgaagtgtcggggccttagttattctactgtaaactctcttgatatttatatacaatctattttgaattaaatattttttaatatttactgcatctgcaaaattatattttagcataaactctctgttgttttctaagctgtagtttctggggaaaaaaaagtgtttctaaacttaatacatttgtaggactcatctccaatataaattccctgatgttgaacaaacttgagcaactgctttaggattttcctccagtacaaaatgtgtgcaataagatctgtgatactagtaaatgtactatgtaactccctttatatttgtaatgcttgtcttcacaataaatactcttcttcactttaaaggcttatacttgctgaaagttttgacagtaattgccattttaatgcttttattaaaaggaagatttttatgttgagttagatgtgagtaggaattaataggttttccatattccttctatttgtacaatttttctcaaggatactagcttttctgtgagataaggtgtaagaactgattaaaagttttgccacattcttcacacttgtaggagttttgccagtatgaattatccaacctacaatcaagagtggcaaccatataaaggctttgtcacattttatatatttctagggtttcacactagtataattattgttatgtgtagagaagttggaggtgttcgtaaaagcaatgtcacattttttagctttgcggatttcctcttcaacatgaattattgccatgcctcttaagaattgagaacttgtggctgggcgtcgtggctcacgcctgtaatcccagcactttaggaggccaaggtgggtggatcacctgaggtcaggagttcgagaccagcctggcaaacatggcgaagtcgcatctctactaaaaataaaaaaattagctgggcatgttggaggacacctgtaatcccagctactcaggaagctgaggtaggagaatggcttaaacccaggaggcagaggttgcagtgagccgagatcatggcactgtactccagcttggatgacaagcatgaaacttcatctcaaaaaaaaaaatattgaaaacttgttataggatttgccacattcctcaaacttgtaggatttttgtccagcatgaattatgtgtaagaagggttcagaacttcctaaaagcgttgtcacattctttatatttgtagggtttatgttccatataaattctcatatttagtaaaagttgatagctggttaaaggctttccgacattcatcaaactcacagggtttctctccagtacgaattatcttatgtctagtaagggcagaggtgtccttaaaggctttgctgcattttcttatttgttgggtttctttcccgcatgaattatctaatgtctactaaggtttgaggatgaaataaaggctttgccacatttatcacacttgtacagtttccctccaatatgaattttcttatgtgaaaaaagcatagtgggatagcttaaagctttgccacattcctcacatttatagtttctctccagtatgaattaccttatgtgtagtaagggtagaggggcacttaaagcctttgccacattcttcacatttgtagggtttctctccagtatgaattctcttatgtctagtaaggataaaggagcgcttaaaagccttgccacatcgttcacatttgtagggtttctctccagtatgaattctcttatgtgcagtaaggtgtgaggacgagttgaaggctttgccacattcttcacatttgtagggtttctctccagtatgaattctcttatgtgtagtaaggatagagaagcacttaaaggccttgccacattcttcacacttgaagggttgctgtccagtatggattatcttatgtgtagtaagggaagaggagtacttaaaggcttcgccacattcttcacatttgtagggtttctctccagtatgaattctcttatgtgtagtaaggtgtgaggaccagttgaaggctttgccacattcttcacatttgtagggtttctctccactatgaattatcttgtgtgtagtaagggatgagaagtacttaaaggctctgccacattcttcacatttgtagggtttctctccagtatgaattcttttatgtgtagtaaggacagaggggtgcttaaaggctttgccacattcttcacatttgtagggtttctctccgctatgaattatcttatgcgcagtaaggatagaggagcgcttaaaggccttgccacattcttcacatttgtagggtttctctccagtatgaattatcttatgtgtagtaaggttagaggagcgcttaaaggccttgccacattcttcacatttgtagggtttctctccactatgaattatcttatgtgcagtaaggtatgaaaaccggctaaaggctttgccacagtcttcacatttgtaccgtttctctccagtatgaattctcttatgtgtagtaaggtgtgaggaccagttgaaggctttgccacattcttcacatttgaagggtttctccccagtatgaattttcttatgtgtagtaagggttgaagactggttaaaagctttgccacattctatacatttgaaaggtttttttccagtatgtcttatcttatgtctgtttgaatttgaaaatttatgaatgactttcacatatttatcacactgaaatattttgctttgagtagttgtcaaatattggttaagtccattataacctcttttgtgcaccttacactcatctacactttcacagccctttttaaactgtaaattgtcatgtccatagttttcatatcttctcagtgtcactttttggaaagaatcttttatgctctgctctggccaaagatctcgggcaaaatgagaacacgtaactgaggggttggctaccatctcatgtttcttcatggtcaaaggtttttttccttgctccagacaggtgatgaggtctggcttagagacaacaataccaaggaagaccaggtttctgtagttctctaacatcacattcctatataaattccgctgtgcagtgtccaggcaatgccactcctccagagagaattctatggccacgtctctaaattgcaatggccccaatgatgtcaatgtttttggcccaagaaggatattttgtcaaacatccagtaagtggaagagcctgtttttcccagtttttctggccatttctaggcttccaggggctcccgggcgtcttagctgtggatctcccaatacctgcaggacacagggccacagaggctgggcctctaggagcagaggacacacagcagtgaagacaagacctggagctccggctgcagagacaaaggccccgcaaaacccggaagccttccgcttcactct

SEQ ID NO: 15875 - RNA, 3847 nt, Homo sapiens
  source 1..3847: mol_type = other RNA
gctgggattacaggcatgagccatcaagcccggccctaacagttttaaaatgcactgcattttattacataaaagtacaagtagtaaagtaatatactcatttattttaatatacttttaattatttctttgtgtcactataataaagtattgctctgaacatttacgttatacattacttaatagaattttactacaaacagcttctccacttgtattttcattatgcgtcttacattttaatgttcttactattttatagaaaaagtcataatgtccaaataatgtaaaaaaatcgaatatctctgatgcagaagccactgatcacatgctttctcacatgtgaatagaaataaaataacagcataatttgaaagctgtattacatcattattcagctttcaaaaaattttattcaaggaaacaagtatactttcaacgtaattacaatgcttccaaaaatctactccttttaaagttaaatagaaatcatttacctaaaaactgcagttgtggattagtttttatattcaatgctctgatttagtgtaatgtctgaagtgtcggggccttagttattctactgtaaactctcttgatatttatatacaatctattttgaattaaatattttttaatatttactgcatctgcaaaattatattttagcataaactctctgttgttttctaagctgtagtttctggggaaaaaaaagtgtttctaaacttaatacatttgtaggactcatctccaatataaattccctgatgttgaacaaacttgagcaactgctttaggattttcctccagtacaaaatgtgtgcaataagatctgtgatactagtaaatgtactatgtaactccctttatatttgtaatgcttgtcttcacaataaatactcttcttcactttaaaggcttatacttgctgaaagttttgacagtaattgccattttaatgcttttattaaaaggaagatttttatgttgagttagatgtgagtaggaattaataggttttccatattccttctatttgtacaatttttctcaaggatactagcttttctgtgagataaggtgtaagaactgattaaaagttttgccacattcttcacacttgtaggagttttgccagtatgaattatccaacctacaatcaagagtggcaaccatataaaggctttgtcacattttatatatttctagggtttcacactagtataattattgttatgtgtagagaagttggaggtgttcgtaaaagcaatgtcacattttttagctttgcggatttcctcttcaacatgaattattgccatgcctcttaagaattgagaacttgtggctgggcgtcgtggctcacgcctgtaatcccagcactttaggaggccaaggtgggtggatcacctgaggtcaggagttcgagaccagcctggcaaacatggcgaagtcgcatctctactaaaaataaaaaaattagctgggcatgttggaggacacctgtaatcccagctactcaggaagctgaggtaggagaatggcttaaacccaggaggcagaggttgcagtgagccgagatcatggcactgtactccagcttggatgacaagcatgaaacttcatctcaaaaaaaaaaatattgaaaacttgttataggatttgccacattcctcaaacttgtaggatttttgtccagcatgaattatgtgtaagaagggttcagaacttcctaaaagcgttgtcacattctttatatttgtagggtttatgttccatataaattctcatatttagtaaaagttgatagctggttaaaggctttccgacattcatcaaactcacagggtttctctccagtacgaattatcttatgtctagtaagggcagaggtgtccttaaaggctttgctgcattttcttatttgttgggtttctttcccgcatgaattatctaatgtctactaaggtttgaggatgaaataaaggctttgccacatttatcacacttgtacagtttccctccaatatgaattttcttatgtgaaaaaagcatagtgggatagcttaaagctttgccacattcctcacatttatagtttctctccagtatgaattaccttatgtgtagtaagggtagaggggcacttaaagcctttgccacattcttcacatttgtagggtttctctccagtatgaattctcttatgtctagtaaggataaaggagcgcttaaaagccttgccacatcgttcacatttgtagggtttctctccagtatgaattctcttatgtgcagtaaggtgtgaggacgagttgaaggctttgccacattcttcacatttgtagggtttctctccagtatgaattctcttatgtgtagtaaggatagagaagcacttaaaggccttgccacattcttcacacttgaagggttgctgtccagtatggattatcttatgtgtagtaagggaagaggagtacttaaaggcttcgccacattcttcacatttgtagggtttctctccagtatgaattctcttatgtgtagtaaggtgtgaggaccagttgaaggctttgccacattcttcacatttgtagggtttctctccactatgaattatcttgtgtgtagtaagggatgagaagtacttaaaggctctgccacattcttcacatttgtagggtttctctccagtatgaattcttttatgtgtagtaaggacagaggggtgcttaaaggctttgccacattcttcacatttgtagggtttctctccgctatgaattatcttatgcgcagtaaggatagaggagcgcttaaaggccttgccacattcttcacatttgtagggtttctctccagtatgaattatcttatgtgtagtaaggttagaggagcgcttaaaggccttgccacattcttcacatttgtagggtttctctccactatgaattatcttatgtgcagtaaggtatgaaaaccggctaaaggctttgccacagtcttcacatttgtaccgtttctctccagtatgaattctcttatgtgtagtaaggtgtgaggaccagttgaaggctttgccacattcttcacatttgaagggtttctccccagtatgaattttcttatgtgtagtaagggttgaagactggttaaaagctttgccacattctatacatttgaaaggtttttttccagtatgtcttatcttatgtctgtttgaatttgaaaatttatgaatgactttcacatatttatcacactgaaatattttgctttgagtagttgtcaaatattggttaagtccattataacctcttttgtgcaccttacactcatctacactttcacagccctttttaaactgtaaattgtcatgtccatagttttcatatcttctcagtgtcactttttggaaagaatcttttatgctctgctctggccaaagatctcgggcaaaatgagaacacgtaactgaggggttggctaccatctcatgtttcttcatggtcaaaggtttttttccttgctccagacaggtgatgaggtctggcttagagacaacaataccaaggaagaccaggtttctgtagttctctaacatcacattcctatataaattccgctgtgcagtgtccaggcaatgccactcctccagagagaattctatggccacgtctctaaattgcaatggccccatttctaggcttccaggggctcccgggcgtcttagctgtggatctcccaatacctgcaggacacagggccacagaggctgggcctctaggagcagaggacacacagcagtgaagacaagacctggagctccggctgcagagac

SEQ ID NO: 15876 - RNA, 3870 nt, Homo sapiens
  source 1..3870: mol_type = other RNA
gctgggattacaggcatgagccatcacacccagccaaaacaaatttcaatgaccttgtctcagaaccttaaggggtctacagctgaattatcttcaggtacccgatgaatccccctaataaaacaggatgaaaaaaattagagtggacataaaatcaaattcaacactactggattatttagagaaaaatgtacttccaacccagtttttcttcagtaactttaactagaaatctttctcgaaaagatggaaaaccagaaggcaacaatctggtagtacaaaaatatacaactaagaaattaccaccaactaggtatgacaactaaatctcattcagaactctgaaaaaaagcatacttggacaaaatactaaactagtggttctcacatcaccaagggtatttatcatgtagaactcctcaaaattacacagggttaggtcaccctgaaaaactaagtcaatgagcctggagtctggctgtatctattctgaaatacctcttcaacaaaatttctaattaggcagcactgtactaaaatgaatgtagtaataacctggattttccatccacatatgggtttgtgtgaaagccactgacagcagtctaacagggtgggagtgtcatggacgctgacgggatcacgtttgtaaggatctctaagatactcaaatggtagacacagggtacctgtgcttggtaaaactacaacttccctactttctgcttaagacatggaggtcagaagcaacccacaatgaactgtgaaccagagatcaaactaaatattccttttaatagaaatgtgaatcttgccatgttgggcagactggtctccaactcctggcttcaagagatcctcccacccgccctagcctcccaaagtgctaggaattacaagtgtgagccaccacatccagccagtgtctttgaaaacaatcaaatataatccttaatgtttctttacattgtcatcaagtattagtaacagtgacttctagtgaacaccttgatccttaaaccacaggtctaagttcagttttgtgattcctttcatttttacactcaaccctgaatatggacaagaccggttagtgtgacctgttattttaggaattacaactttaaaaattcctaatagccacaatctaaatgtgcaattcaaagcttttaacaatttccatgttctaaagtttctaagagtcttgaggttatgctagggctcctggttaaagtaactgccaactgggactgtatgtcacctaagtcaggataactccctggtgaagttacttttatttcaggttctgtattatttctcttagccatattatacccgtaactgtcctttttacagaaacccttccaacttaagagcctgcaaggaagtcatatactgcccaaaaatgcccacataagttgtccatttataaaaagcaatgtaattgacatattgcatggcttccgtaacttcttagctatcttggcttgttcctaacaggaacaggttgtaggctatgtgagaatactaaagacaaaatgcccaatgccagagctctcagtaaataaacaggctgtctgaaaagtgtctttcttgaacatgcttaactttaaggctgaaccttcctgacaccaattctcccaagatttgtgtaaaaggtggaaataaataatttgtttaggaactgtatcttaatgtatccatttagcttgaactcttaatgcaatgacttatctttcatatttaagacagtcaataccgcataatccaaaactatcttaagagcatatttaaggaaactaagccacaagactgttgcattatgatttaatctaattgcacaaaaatttgaaattacaacacctgccattttctaagaggaaggttatgcatgcctccatattcaattctgcactgttacatttgaaccatattgtgaacttttacatcatgatggatcagcttagaattcccatgcaacacctcaaattataaaatggaagcaatttttagacctgtggaaagttttcatgctaaagataaaagccatttgttaatgggcaacttactttgtgtttaagaaccaggttgctgctatactttaaaatgttggtcactaaatattatggaccctgaactggcttctatgcctaaaaaaaaaaaaaatgggttaactatcacttaggtgacatctatatttccttcacttcagaagactaatccatagtgcctctcagctgtttcttataaaataagaatcgtgtaaccaactgcttcccatgggataagaacaatggtaacagtgggttcaactgactatacacaattatgctaatattttattaattcaaaagcactttacaagaaaatataagtatggcttccaataggaatgttatacctggacttggtaccaagctcacagatttgagtttgcaaggaaaaacaggctttcaagttaaagaacaatttgtaaccaaaactttaatcccaaggattctcacaaaacatattacaaatgacagcatgaaaaaaaaatcttgcacagtaactcaaagttcggctctacaatgtacccttaaactggcaggacatttttgaaatcacaaatttgcacataaagaatgtcacgaacagccatgtatccatatacagcaatcaaataaggaacttatgacctaaagcaaaggtaaactttcttgaaacttaacattctataccaactaggcaacctctgcccaggatgagagttggatttttcaaaaacctctaatttaatagtgcagcatttcgttttccctgatggcctgtgtttcacagcagtttttaaagactgcttgttcaactatagctgcagcctatatcccagctatggaaaaaaaagtaaatcttagttcaatttttgccagttgtttctgtatttaaatttaaaaaaaaacacacttccgctgggcaggtttagaggtttattatcagtctgtgcataactaaaagttcaaagcaaattcaattttgcttaagggaacattgtaaagtaacaattcttggtattacatgcctcgtatgatccatttcaaaccatagagaattacacctttgtgtcactgtttcaagagacaaacagatttgaacagctaaaacatcttaaaaatgcaccaagcttatgaagtctcaaacaaaacttgaattttctgtacatactcctgtcaaatgaagtaatttcctgtacaccacttctcttgcaaactgtcttctatttcctttcatttgacctagatcgactacgagacctagagaaggatcgggacggcttgtgatttctctcccgagacagcgatctctctcttctcctatctctagaaagggacctgctccggctgcgagagaagcttctccttcttggagatctgcgacgaggtggaggactcctcctacgataatcatctcgagggcgacgaccccaagagggaggtgggccacgatttctacttcttttttcaccattcgacagttccactcttacacggcagccacatagtgttcttccatctagctctcggactgcatcagctgcatctcggggatcttcaaattcaacaaaagcaaagccgggtgggtttctagcaacccacacacttcggagtggtccatagtagccaaaagcccgttccaattccgtcttgttgccattgtttccaagattgcctacataaaccttacagtccaatggacaggaatcacgatgcatttcgagatctagggttaaaaaatgcggcggctcaaatccacacgctccgatgagtcttcccgctttcctccggcccaacaccaaccaactctctcactcacccggcgtccacgaaatggcgg

SEQ ID NO: 15877 - RNA, 4326 nt, Homo sapiens
  source 1..4326: mol_type = other RNA
gctgggattacaggcatgagccatcacacccagccaaaacaaatttcaatgaccttgtctcagaaccttaaggggtctacagctgaattatcttcaggtacccgatgaatccccctaataaaacaggatgaaaaaaattagagtggacataaaatcaaattcaacactactggattatttagagaaaaatgtacttccaacccagtttttcttcagtaactttaactagaaatctttctcgaaaagatggaaaaccagaaggcaacaatctggtagtacaaaaatatacaactaagaaattaccaccaactaggtatgacaactaaatctcattcagaactctgaaaaaaagcatacttggacaaaatactaaactagtggttctcacatcaccaagggtatttatcatgtagaactcctcaaaattacacagggttaggtcaccctgaaaaactaagtcaatgagcctggagtctggctgtatctattctgaaatacctcttcaacaaaatttctaattaggcagcactgtactaaaatgaatgtagtaataacctggattttccatccacatatgggtttgtgtgaaagccactgacagcagtctaacagggtgggagtgtcatggacgctgacgggatcacgtttgtaaggatctctaagatactcaaatggtagacacagggtacctgtgcttggtaaaactacaacttccctactttctgcttaagacatggaggtcagaagcaacccacaatgaactgtgaaccagagatcaaactaaatattccttttaatagaaatgtgaatcttgccatgttgggcagactggtctccaactcctggcttcaagagatcctcccacccgccctagcctcccaaagtgctaggaattacaagtgtgagccaccacatccagccagtgtctttgaaaacaatcaaatataatccttaatgtttctttacattgtcatcaagtattagtaacagtgacttctagtgaacaccttgatccttaaaccacaggtctaagttcagttttgtgattcctttcatttttacactcaaccctgaatatggacaagaccggttagtgtgacctgttattttaggaattacaactttaaaaattcctaatagccacaatctaaatgtgcaattcaaagcttttaacaatttccatgttctaaagtttctaagagtcttgaggttatgctagggctcctggttaaagtaactgccaactgggactgtatgtcacctaagtcaggataactccctggtgaagttacttttatttcaggttctgtattatttctcttagccatattatacccgtaactgtcctttttacagaaacccttccaacttaagagcctgcaaggaagtcatatactgcccaaaaatgcccacataagttgtccatttataaaaagcaatgtaattgacatattgcatggcttccgtaacttcttagctatcttggcttgttcctaacaggaacaggttgtaggctatgtgagaatactaaagacaaaatgcccaatgccagagctctcagtaaataaacaggctgtctgaaaagtgtctttcttgaacatgcttaactttaaggctgaaccttcctgacaccaattctcccaagatttgtgtaaaaggtggaaataaataatttgtttaggaactgtatcttaatgtatccatttagcttgaactcttaatgcaatgacttatctttcatatttaagacagtcaataccgcataatccaaaactatcttaagagcatatttaaggaaactaagccacaagactgttgcattatgatttaatctaattgcacaaaaatttgaaattacaacacctgccattttctaagaggaaggttatgcatgcctccatattcaattctgcactgttacatttgaaccatattgtgaacttttacatcatgatggatcagcttagaattcccatgcaacacctcaaattataaaatggaagcaatttttagacctgtggaaagttttcatgctaaagataaaagccatttgttaatgggcaacttactttgtgtttaagaaccaggttgctgctatactttaaaatgttggtcactaaatattatggaccctgaactggcttctatgcctaaaaaaaaaaaaaatgggttaactatcacttaggtgacatctatatttccttcacttcagaagactaatccatagtgcctctcagctgtttcttataaaataagaatcgtgtaaccaactgcttcccatgggataagaacaatggtaacagtgggttcaactgactatacacaattatgctaatattttattaattcaaaagcactttacaagaaaatataagtatggcttccaataggaatgttatacctggacttggtaccaagctcacagatttgagtttgcaaggaaaaacaggctttcaagttaaagaacaatttgtaaccaaaactttaatcccaaggattctcacaaaacatattacaaatgacagcatgaaaaaaaaatcttgcacagtaactcaaagttcggctctacaatgtacccttaaactggcaggacatttttgaaatcacaaatttgcacataaagaatgtcacgaacagccatgtatccatatacagcaatcaaataaggaacttatgacctaaagcaaaggtaaactttcttgaaacttaacattctataccaactaggcaacctctgcccaggatgagagttggatttttcaaaaacctctaatttaatagtgcagcatttcgttttccctgatggcctgtgtttcacagcagtttttaaagactgcttgttcaactatagctgcagcctatatcccagctatggaaaaaaaagtaaatcttagttcaatttttgccagttgtttctgtatttaaatttaaaaaaaaacacacttccgctgggcaggtttagaggtttattatcagtctgtgcataactaaaagttcaaagcaaattcaattttgcttaagggaacattgtaaagtaacaattcttggtattacatgcctcgtatgatccatttcaaaccatagagaattacacctttgtgtcactgtttcaagagacaaacagatttgaacagctaaaacatcttaaaaatgcaccaagcttatgaagtctcaaacaaaacttgaattttctgtacatactcctgtcaaatgaagtaatttcctgtacaccacttctcttgcaaactgtcttctatttcctttcatttgacctagatcgactacgagacctagagaaggatcgggacggcttgtgatttctctcccgagacagcgatctctctcttctcctatctctagaaagggacctgctccggctgcgagagaagcttctccttcttggagattagttttgggtttcaacaagctagaaatggtgaggtgaggctgccggactgacggccaggaagaatttgctgaaaaggttttgccagatgttgcgttggatttagttggttggcgaagggggtgttgtggatttttcctgcttttttgttagccgaaggctgctgctgtagttgttgtgaagacatttggtaaataaacagctgagctgattggccaggaatgtgtgggcggtcgaggtggctgctgccgatttggttaaggttggagagaaggctgagagaaaacagcatgctcgggaaccaaagggcggtgcaacctgacgactggccagcctgggtcatgtgaaacgacaccagccaagctgaatggggcgcgctggtcacatgacgctgaaagggctagttgactggctaatgcagattcagagggtggtgagaagagacatgatggtgactctgcgacgaggtggaggactcctcctacgataatcatctcgagggcgacgaccccaagagggaggtgggccacgatttctacttcttttttcaccattcgacagttccactcttacacggcagccacatagtgttcttccatctagctctcggactgcatcagctgcatctcggggatcttcaaattcaacaaaagcaaagccgggtgggtttctagcaacccacacacttcggagtggtccatagtagccaaaagcccgttccaattccgtcttgttgccattgtttccaagattgcctacataaaccttacagtccaatggacaggaatcacgatgcatttcgagatctagggttaaaaaatgcggcggctcaaatccacacgctccgatgagtcttcccgctttcctccggcccaacaccaaccaactctctcactcacccggcgtccacgaaatggcgg

SEQ ID NO: 15878 - RNA, 2342 nt, Homo sapiens
  source 1..2342: mol_type = other RNA
gctgggattacaggcatgagccatcacacccagcccatgtgtgttttcttattctttaaaaagaacactttgaggctgggcgtggtggctcatgcctgtaatcccagcactttgggaggccgagacagacagatcacttgagatcaggagttcaagaccagcctggccaacatggcaaaaccccatctctactaaaaaatacaaaaattagccaggcatggtggtgcatgtctatagtcccagctactcgggaggctgatgcatgagaattgcttgaaccctggaggcagaggctgggagtcagaggttgcagtgagctgagatcgtcccactgtactccagcctgggcaacacagcaagacattgtctcaaaaagaaaaaaaaagaaaaaaaagatccgtttgagtgcattgtgggaaatggatttaaaggtagcaaaaataaatacaggaaaacctgtttgaaagctatattagtaatcagagtgagatgaatcagaccaaggtgacaacattaaagataaaaaacagtataaattctagaaacatttaggactcaggatctataggacttggtgattgactgggttgggtggtgacagtgactccccaatgtgaattctctggtgatgagcaaggtgtgcatgctgcctgaaggtttttttgcattccttacattcatagggtctctctccagtatgaattctctgatgttgggcaagggatccacagtaactaaaagcctttccacaaacagtacattcataaggtttctctccagtatgaactcgctgatgttgagtaagggacgagtcattgctaaaagccttcccacattcaatacattcatagggtttctctccagtatgaactctttgatgctgagcaaggtaggcaatctggctgaatgctttcctacattcctgacacttataaggtttttctccagtatgaattctctgatgttgagcaaggtgtgaattctggctaaaggccttcccacattccttacattcatagggtctctctccagtatgtattctctgatgtacagtaaggtatgcacgaaggctaaatgctttcccacagacattacattcatagggtttctctcctgtatgaactctctggtgttgagcaatggatgatctgttgctaaatgctttcccacattcgatacattcatagggtttctctcccgtgtgaactctctgatgttgagcaaggtaggcaaactggctgaaggcttttcgacataccttacattcgtaaggtttttctccagtatgaactcgcagatgttgaactaggtgtgcattctgactgaaggctttcctacattccttacattcatagggtttttctccagtatgaatcctctgatgttgaacaagatttgatctctggctgaaggcttttccacactctatacatttatagggtttctctccagtatgaattctttgatgaagagtaagggatgaactctggctgaagactttttcacagtcattacatttcaaaagtttcttctctgcacagacactcttgggcttaatagccattaaattttttttaaagcttctcttttgtgtgtcatgtttatgtactttctcctctttggggattatcttttgtgtacaaagcagtgggttctgatgaaaacttccccaagatttatattcttgttctctctcatcaaaaaggggttcttcatgagtgattatctcttccttgaaacacgccttctgattacctggttgcctttcaaaatagccctcacatttccactcttctctcaaactggagtattcaaggttatagcttgtaagtgtttctattatcttctgggattgatgttcttcataaaaatcctgctttggggttaattcttcagtctcacatataggctcccagcctgagcacaagccttttgtcagctctctcttcaccatccagggtgcttttccttgttccaacaataatatcacacttggtttggaaaagcaaagtcccagtgataccaagatcctgtagttctctagcatcacattactgtacagatgtctttgagaagaatccagacaatcccattcctcttgggagaagtctacagccacatctctgaaggtcaccaactcctccactcgcaccggagtcacacagatggcctgcgacgagcttccggagacccacacgccactcctcagcccactcccgacctgcagaacagaactggtggaagatctccttcctgccccgaaggctcggggaatctgcactcgggtctcaccgctacccttagttggatggaacccagcccttacgggcccggaaagaagc

SEQ ID NO: 15879 - RNA, 2309 nt, Homo sapiens
  source 1..2309: mol_type = other RNA
gctgggattacaggcatgagccatcacacccagcccatgtgtgttttcttattctttaaaaagaacactttgaggctgggcgtggtggctcatgcctgtaatcccagcactttgggaggccgagacagacagatcacttgagatcaggagttcaagaccagcctggccaacatggcaaaaccccatctctactaaaaaatacaaaaattagccaggcatggtggtgcatgtctatagtcccagctactcgggaggctgatgcatgagaattgcttgaaccctggaggcagaggctgggagtcagaggttgcagtgagctgagatcgtcccactgtactccagcctgggcaacacagcaagacattgtctcaaaaagaaaaaaaaagaaaaaaaagatccgtttgagtgcattgtgggaaatggatttaaaggtagcaaaaataaatacaggaaaacctgtttgaaagctatattagtaatcagagtgagatgaatcagaccaaggtgacaacattaaagataaaaaacagtataaattctagaaacatttaggactcaggatctataggacttggtgattgactgggttgggtggtgacagtgactccccaatgtgaattctctggtgatgagcaaggtgtgcatgctgcctgaaggtttttttgcattccttacattcatagggtctctctccagtatgaattctctgatgttgggcaagggatccacagtaactaaaagcctttccacaaacagtacattcataaggtttctctccagtatgaactcgctgatgttgagtaagggacgagtcattgctaaaagccttcccacattcaatacattcatagggtttctctccagtatgaactctttgatgctgagcaaggtaggcaatctggctgaatgctttcctacattcctgacacttataaggtttttctccagtatgaattctctgatgttgagcaaggtgtgaattctggctaaaggccttcccacattccttacattcatagggtctctctccagtatgtattctctgatgtacagtaaggtatgcacgaaggctaaatgctttcccacagacattacattcatagggtttctctcctgtatgaactctctggtgttgagcaatggatgatctgttgctaaatgctttcccacattcgatacattcatagggtttctctcccgtgtgaactctctgatgttgagcaaggtaggcaaactggctgaaggcttttcgacataccttacattcgtaaggtttttctccagtatgaactcgcagatgttgaactaggtgtgcattctgactgaaggctttcctacattccttacattcatagggtttttctccagtatgaatcctctgatgttgaacaagatttgatctctggctgaaggcttttccacactctatacatttatagggtttctctccagtatgaattctttgatgaagagtaagggatgaactctggctgaagactttttcacagtcattacatttcaaaagtttcttctctgcacagacactcttgggcttaatagccattaaattttttttaaagcttctcttttgtgtgtcatgtttatgtactttctcctctttggggattatcttttgtgtacaaagcagtgggttctgatgaaaacttccccaagatttatattcttgttctctctcatcaaaaaggggttcttcatgagtgattatctcttccttgaaacacgccttctgattacctggttgcctttcaaaatagccctcacatttccactcttctctcaaactggagtattcaaggttatagcttgtaagtgtttctattatcttctgggattgatgttcttcataaaaatcctgctttggggttaattcttcagtctcacatataggctcccagcctgagcacaagccttttgtcagctctctcttcaccatccagggtgcttttccttgttccaacaataatatcacacttggtttggaaaagcaaagtcccagtgataccaagatcctgtagttctctagcatcacattactgtacagatgtctttgagaagaatccagacaatcccattcctcttgggagaagtctacagccacatctctgaaggtcaccaactcctggtacatggctttaagaagcccaacagccattctttcttcctcctggctcttctcttgggaaatagcagtggcctcagatgaagcctcacattccacggtgccattgacttcctcgcacccagtcacacaggacgtggacaggcacacggggtgacagcctcgcact

SEQ ID NO: 15880 - RNA, 2460 nt, Homo sapiens
  source 1..2460: mol_type = other RNA
gctgggattacaggcatgagccatcacacccagcccatgtgtgttttcttattctttaaaaagaacactttgaggctgggcgtggtggctcatgcctgtaatcccagcactttgggaggccgagacagacagatcacttgagatcaggagttcaagaccagcctggccaacatggcaaaaccccatctctactaaaaaatacaaaaattagccaggcatggtggtgcatgtctatagtcccagctactcgggaggctgatgcatgagaattgcttgaaccctggaggcagaggctgggagtcagaggttgcagtgagctgagatcgtcccactgtactccagcctgggcaacacagcaagacattgtctcaaaaagaaaaaaaaagaaaaaaaagatccgtttgagtgcattgtgggaaatggatttaaaggtagcaaaaataaatacaggaaaacctgtttgaaagctatattagtaatcagagtgagatgaatcagaccaaggtgacaacattaaagataaaaaacagtataaattctagaaacatttaggactcaggatctataggacttggtgattgactgggttgggtggtgacagtgactccccaatgtgaattctctggtgatgagcaaggtgtgcatgctgcctgaaggtttttttgcattccttacattcatagggtctctctccagtatgaattctctgatgttgggcaagggatccacagtaactaaaagcctttccacaaacagtacattcataaggtttctctccagtatgaactcgctgatgttgagtaagggacgagtcattgctaaaagccttcccacattcaatacattcatagggtttctctccagtatgaactctttgatgctgagcaaggtaggcaatctggctgaatgctttcctacattcctgacacttataaggtttttctccagtatgaattctctgatgttgagcaaggtgtgaattctggctaaaggccttcccacattccttacattcatagggtctctctccagtatgtattctctgatgtacagtaaggtatgcacgaaggctaaatgctttcccacagacattacattcatagggtttctctcctgtatgaactctctggtgttgagcaatggatgatctgttgctaaatgctttcccacattcgatacattcatagggtttctctcccgtgtgaactctctgatgttgagcaaggtaggcaaactggctgaaggcttttcgacataccttacattcgtaaggtttttctccagtatgaactcgcagatgttgaactaggtgtgcattctgactgaaggctttcctacattccttacattcatagggtttttctccagtatgaatcctctgatgttgaacaagatttgatctctggctgaaggcttttccacactctatacatttatagggtttctctccagtatgaattctttgatgaagagtaagggatgaactctggctgaagactttttcacagtcattacatttcaaaagtttcttctctgcacagacactcttgggcttaatagccattaaattttttttaaagcttctcttttgtgtgtcatgtttatgtactttctcctctttggggattatcttttgtgtacaaagcagtgggttctgatgaaaacttccccaagatttatattcttgttctctctcatcaaaaaggggttcttcatgagtgattatctcttccttgaaacacgccttctgattacctggttgcctttcaaaatagccctcacatttccactcttctctcaaactggagtattcaaggttatagcttgtaagtgtttctattatcttctgggattgatgttcttcataaaaatcctgctttggggttaattcttcagtctcacatataggctcccagcctgagcacaagccttttgtcagctctctcttcaccatccagggtgcttttccttgttccaacaataatatcacacttggtttggaaaagcaaagtcccagtgataccaagatcctgtagttctctagcatcacattactgtacagatgtctttgagaagaatccagacaatcccattcctcttgggagaagtctacagccacatctctgaaggtcaccaactcctggtacatggctttaagaagcccaacagccattctttcttcctcctggctcttctcttgggaaatagcagtggcctcagatgactccactcgcaccggagtcacacagatggcctgcgacgagcttccggagacccacacgccactcctcagcccactcccgacaatcgagaagtccagaaagaacaaatacatgcacattgtctctgacaaaactgcaaggtcagaatcaaacagccacgagaatataaaacgcgaccatggtcacacaaaaggtcgcatattcgcacgacctcagatgtcactggacagggtctctc

SEQ ID NO: 15881 - RNA, 2426 nt, Homo sapiens
  source 1..2426: mol_type = other RNA
gctgggattacaggcatgagccatcacacccagcccatgtgtgttttcttattctttaaaaagaacactttgaggctgggcgtggtggctcatgcctgtaatcccagcactttgggaggccgagacagacagatcacttgagatcaggagttcaagaccagcctggccaacatggcaaaaccccatctctactaaaaaatacaaaaattagccaggcatggtggtgcatgtctatagtcccagctactcgggaggctgatgcatgagaattgcttgaaccctggaggcagaggctgggagtcagaggttgcagtgagctgagatcgtcccactgtactccagcctgggcaacacagcaagacattgtctcaaaaagaaaaaaaaagaaaaaaaagatccgtttgagtgcattgtgggaaatggatttaaaggtagcaaaaataaatacaggaaaacctgtttgaaagctatattagtaatcagagtgagatgaatcagaccaaggtgacaacattaaagataaaaaacagtataaattctagaaacatttaggactcaggatctataggacttggtgattgactgggttgggtggtgacagtgactccccaatgtgaattctctggtgatgagcaaggtgtgcatgctgcctgaaggtttttttgcattccttacattcatagggtctctctccagtatgaattctctgatgttgggcaagggatccacagtaactaaaagcctttccacaaacagtacattcataaggtttctctccagtatgaactcgctgatgttgagtaagggacgagtcattgctaaaagccttcccacattcaatacattcatagggtttctctccagtatgaactctttgatgctgagcaaggtaggcaatctggctgaatgctttcctacattcctgacacttataaggtttttctccagtatgaattctctgatgttgagcaaggtgtgaattctggctaaaggccttcccacattccttacattcatagggtctctctccagtatgtattctctgatgtacagtaaggtatgcacgaaggctaaatgctttcccacagacattacattcatagggtttctctcctgtatgaactctctggtgttgagcaatggatgatctgttgctaaatgctttcccacattcgatacattcatagggtttctctcccgtgtgaactctctgatgttgagcaaggtaggcaaactggctgaaggcttttcgacataccttacattcgtaaggtttttctccagtatgaactcgcagatgttgaactaggtgtgcattctgactgaaggctttcctacattccttacattcatagggtttttctccagtatgaatcctctgatgttgaacaagatttgatctctggctgaaggcttttccacactctatacatttatagggtttctctccagtatgaattctttgatgaagagtaagggatgaactctggctgaagactttttcacagtcattacatttcaaaagtttcttctctgcacagacactcttgggcttaatagccattaaattttttttaaagcttctcttttgtgtgtcatgtttatgtactttctcctctttggggattatcttttgtgtacaaagcagtgggttctgatgaaaacttccccaagatttatattcttgttctctctcatcaaaaaggggttcttcatgagtgattatctcttccttgaaacacgccttctgattacctggttgcctttcaaaatagccctcacatttccactcttctctcaaactggagtattcaaggttatagcttgtaagtgtttctattatcttctgggattgatgttcttcataaaaatcctgctttggggttaattcttcagtctcacatataggctcccagcctgagcacaagccttttgtcagctctctcttcaccatccagggtgcttttccttgttccaacaataatatcacacttggtttggaaaagcaaagtcccagtgataccaagatcctgtagttctctagcatcacattactgtacagatgtctttgagaagaatccagacaatcccattcctcttgggagaagtctacagccacatctctgaaggtcaccaactcctggtacatggctttaagaagcccaacagccattctttcttcctcctggctcttctcttgggaaatagcagtggcctcagatgactccactcgcaccggagtcacacagatggcctgcgacgagcttccggagacccacacgccactcctcagcccactcccgacctgcagaacagaactggtggaagatctccttcctgccccgaaggctcggggaatctgcactcgggtctcaccgctacccttagttggatggaacccagcccttacgggcccggaaagaagc

SEQ ID NO: 15882 - RNA, 2401 nt, Homo sapiens
  source 1..2401: mol_type = other RNA
gctgggattacaggcatgagccatcacacccagcccatgtgtgttttcttattctttaaaaagaacactttgaggctgggcgtggtggctcatgcctgtaatcccagcactttgggaggccgagacagacagatcacttgagatcaggagttcaagaccagcctggccaacatggcaaaaccccatctctactaaaaaatacaaaaattagccaggcatggtggtgcatgtctatagtcccagctactcgggaggctgatgcatgagaattgcttgaaccctggaggcagaggctgggagtcagaggttgcagtgagctgagatcgtcccactgtactccagcctgggcaacacagcaagacattgtctcaaaaagaaaaaaaaagaaaaaaaagatccgtttgagtgcattgtgggaaatggatttaaaggtagcaaaaataaatacaggaaaacctgtttgaaagctatattagtaatcagagtgagatgaatcagaccaaggtgacaacattaaagataaaaaacagtataaattctagaaacatttaggactcaggatctataggacttggtgattgactgggttgggtggtgacagtgactccccaatgtgaattctctggtgatgagcaaggtgtgcatgctgcctgaaggtttttttgcattccttacattcatagggtctctctccagtatgaattctctgatgttgggcaagggatccacagtaactaaaagcctttccacaaacagtacattcataaggtttctctccagtatgaactcgctgatgttgagtaagggacgagtcattgctaaaagccttcccacattcaatacattcatagggtttctctccagtatgaactctttgatgctgagcaaggtaggcaatctggctgaatgctttcctacattcctgacacttataaggtttttctccagtatgaattctctgatgttgagcaaggtgtgaattctggctaaaggccttcccacattccttacattcatagggtctctctccagtatgtattctctgatgtacagtaaggtatgcacgaaggctaaatgctttcccacagacattacattcatagggtttctctcctgtatgaactctctggtgttgagcaatggatgatctgttgctaaatgctttcccacattcgatacattcatagggtttctctcccgtgtgaactctctgatgttgagcaaggtaggcaaactggctgaaggcttttcgacataccttacattcgtaaggtttttctccagtatgaactcgcagatgttgaactaggtgtgcattctgactgaaggctttcctacattccttacattcatagggtttttctccagtatgaatcctctgatgttgaacaagatttgatctctggctgaaggcttttccacactctatacatttatagggtttctctccagtatgaattctttgatgaagagtaagggatgaactctggctgaagactttttcacagtcattacatttcaaaagtttcttctctgcacagacactcttgggcttaatagccattaaattttttttaaagcttctcttttgtgtgtcatgtttatgtactttctcctctttggggattatcttttgtgtacaaagcagtgggttctgatgaaaacttccccaagatttatattcttgttctctctcatcaaaaaggggttcttcatgagtgattatctcttccttgaaacacgccttctgattacctggttgcctttcaaaatagccctcacatttccactcttctctcaaactggagtattcaaggttatagcttgtaagtgtttctattatcttctgggattgatgttcttcataaaaatcctgctttggggttaattcttcagtctcacatataggctcccagcctttgagtcaagctgagctgtcacgtgcaaagatttttgccaatttcctcttcactaacctgagcacaagccttttgtcagctctctcttcaccatccagggtgcttttccttgttccaacaataatatcacacttggtttggaaaagcaaagtcccagtgataccaagatcctgtagttctctagcatcacattactgtacagatgtctttgagaagaatccagacaatcccattcctcttgggagaagtctacagccacatctctgaaggtcaccaactcctccactcgcaccggagtcacacagatggcctgcgacgagcttccggagacccacacgccactcctcagcccactcccgacctgcagaacagaactggtggaagatctccttcctgccccgaaggctcggggaatctgcactcgggtctcaccgctacccttagttggatggaacccagcccttacgggcccggaaagaagc

SEQ ID NO: 15883 - RNA, 2485 nt, Homo sapiens
  source 1..2485: mol_type = other RNA
gctgggattacaggcatgagccatcacacccagcccatgtgtgttttcttattctttaaaaagaacactttgaggctgggcgtggtggctcatgcctgtaatcccagcactttgggaggccgagacagacagatcacttgagatcaggagttcaagaccagcctggccaacatggcaaaaccccatctctactaaaaaatacaaaaattagccaggcatggtggtgcatgtctatagtcccagctactcgggaggctgatgcatgagaattgcttgaaccctggaggcagaggctgggagtcagaggttgcagtgagctgagatcgtcccactgtactccagcctgggcaacacagcaagacattgtctcaaaaagaaaaaaaaagaaaaaaaagatccgtttgagtgcattgtgggaaatggatttaaaggtagcaaaaataaatacaggaaaacctgtttgaaagctatattagtaatcagagtgagatgaatcagaccaaggtgacaacattaaagataaaaaacagtataaattctagaaacatttaggactcaggatctataggacttggtgattgactgggttgggtggtgacagtgactccccaatgtgaattctctggtgatgagcaaggtgtgcatgctgcctgaaggtttttttgcattccttacattcatagggtctctctccagtatgaattctctgatgttgggcaagggatccacagtaactaaaagcctttccacaaacagtacattcataaggtttctctccagtatgaactcgctgatgttgagtaagggacgagtcattgctaaaagccttcccacattcaatacattcatagggtttctctccagtatgaactctttgatgctgagcaaggtaggcaatctggctgaatgctttcctacattcctgacacttataaggtttttctccagtatgaattctctgatgttgagcaaggtgtgaattctggctaaaggccttcccacattccttacattcatagggtctctctccagtatgtattctctgatgtacagtaaggtatgcacgaaggctaaatgctttcccacagacattacattcatagggtttctctcctgtatgaactctctggtgttgagcaatggatgatctgttgctaaatgctttcccacattcgatacattcatagggtttctctcccgtgtgaactctctgatgttgagcaaggtaggcaaactggctgaaggcttttcgacataccttacattcgtaaggtttttctccagtatgaactcgcagatgttgaactaggtgtgcattctgactgaaggctttcctacattccttacattcatagggtttttctccagtatgaatcctctgatgttgaacaagatttgatctctggctgaaggcttttccacactctatacatttatagggtttctctccagtatgaattctttgatgaagagtaagggatgaactctggctgaagactttttcacagtcattacatttcaaaagtttcttctctgcacagacactcttgggcttaatagccattaaattttttttaaagcttctcttttgtgtgtcatgtttatgtactttctcctctttggggattatcttttgtgtacaaagcagtgggttctgatgaaaacttccccaagatttatattcttgttctctctcatcaaaaaggggttcttcatgagtgattatctcttccttgaaacacgccttctgattacctggttgcctttcaaaatagccctcacatttccactcttctctcaaactggagtattcaaggttatagcttgtaagtgtttctattatcttctgggattgatgttcttcataaaaatcctgctttggggttaattcttcagtctcacatataggctcccagcctttgagtcaagctgagctgtcacgtgcaaagatttttgccaatttcctcttcactaacctgagcacaagccttttgtcagctctctcttcaccatccagggtgcttttccttgttccaacaataatatcacacttggtttggaaaagcaaagtcccagtgataccaagatcctgtagttctctagcatcacattactgtacagatgtctttgagaagaatccagacaatcccattcctcttgggagaagtctacagccacatctctgaaggtcaccaactcctggtacatggctttaagaagcccaacagccattctttcttcctcctggctcttctcttgggaaatagcagtggcctcagatgactccactcgcaccggagtcacacagatggcctgcgacgagcttccggagacccacacgccactcctcagcccactcccgacctgcagaacagaactggtggaagatctccttcctgccccgaaggctcggggaatctgcactcgggtctcaccgctacccttagttggatggaacccagcccttacgggcccggaaagaagc

SEQ ID NO: 15884 - RNA, 10256 nt, Homo sapiens
  source 1..10256: mol_type = other RNA
gctgggattacaggcatgagccatcacacccagcctctgtgtttcattttttatctctggggatgagcacaagccagagctctattctaccaagctactatttggattgtacaatatcgtgattcttagaatgtaatgaaaaaggaaagccctttcttcacatgaaatctgctgaagaaggtctccttgtaaagcagataagagctggcagaaggcaggacagcttgaggccaggtcgcccatctccagtctctccctccaccctgggacctcttctcacccctagaatctccccctcccggcctcttcccctaagtctcttcctccattcccagacacctatggttccaactggccaggtacatccgggccacttaaagggccctgttaagctgcagagttgagagcagtgtgagaatctctgcttccttagcaggtggaattccattcttttgaagccaagggaggcaaaaaagcagagacggttcttatgatttccttgactgactgataagtttcccagacacgctattccccacggtggacttgacggccgcaaaccctatgggattcaggttacctgaacacgatctcatatttccccacattcctccacacggcggacttgatggccttacatctgatgggattccagttacctgaacgcgatctcatatttcccacggttcttcaattgcaggggctgcttcgcctcctctgtgaccctgacaatcccaaaatccagtcccccttcagctcctttggggaaggtgatgtccaaggcgatgtcgtatgcctctgcaaagaccatgatattttcaatctgaacaacaccaagaagattttctgcatctaaaacctccaaccgaatagccttcttgatgttgacaggcttggtgggctgaaagtacaggtgcaggccgtactcagcctcaggggggatggtcccctgcatcagggatacagtgaaatcatcacccaagtgctccaggctggtgatccgccaggccacaggcaggagcgtgacattgcggagaagaactaccctggattcctgtctgtgcagcaagagccggtcaaaatgtaattgcctgggttccagctctagttccgggcggatcccctggcagcttaattggaagatggctggctctgggttgtcattgatgcagcagacaatgctgtcttcaaagacaccaactgaagtagggtaggcccatacgtttaatatctgcttctcattgggtttcaggaccatggtgttgggttccaggaagtacgtgtttgctttgacatcattctgaaaatagaaggatgcctccaccaccattaaggaagtgttcaggattgttagcgtctccatgttgcctgggaataaggatgacttgtacttatctcttgattttccacaaagtagtggcccaaagtagtacgtctccgtgctcataacatacttcttaaagatgacctcatttgtcttcatgtccatcttccgctgaggaaataccacttttgggtcttggcaaatgtatgggtaagtgcagatgcctcggcagtagagctggtactggcagcaagttcctaggatctcaaagttaaaggtttggtcaaagttcccgaactcatcagaagagaagtgcacctgcaacgttacctcgccattggctggcacgatccaccggaagtgattcagtctggtgaatttctcctgggagtgctgcccgttgaagttgtccaggtctgtatctgacagctgggaaatggttccagcaggttccccagaaaggaccttcctgtttaaggccatgtgacgcttgtctttctgactctcgaagacttggtctatcttttctttcattttctgtttgccccccttagatgagctggtctgctcctcttgagcctgctctcctttgggaagcctgtcgctctctagggcctgcttccagctcaagccttcaaagtctggtgtctggatgttaaggaagggtacgcccaggtccttctccttcttctcttcgtggtcctcctccccttccccctcccagtcgctccgctcctccagggctcgcagcttctccaggcgctcccgctccgccttctccctctccaggcgctccttctccaggcgctctctctcccggtccttgcggcccctgcgcccacccgaggggacctggcgctggtcgtcgggctcatggggagcttcctccatccctgcaggaggcagctggactccttgcttccggtcccagtacatgaggatgttctggacatccttcagtgtcaattcataggtcttaaacttctgggccagttgcttgtcggggtcctttgagatgtccccttcactgtcctcttggtcctggacaagaggaagcccatgcatgctgacatcgcccatgttccttttcttcttatttagctcttccttctcagacattgtttgttccctaacagatattttcctttcgattgtctccatcttgacatccactttggtgagcggaggaactgtgctgcattccagcttcctcatctccaaaatgatggtgatgatcatatctccctcagcgggtgttgtggagactggagatagatggtgatgggatctattcacagttcccagcagggagtgtcacatagcaggaattcagcacacagtagctgcttgtttgctgcttgagatttcttcatggggggctcctccttaatgggtccctgctttccttttttgaccctccgtttcagctcatcctcttccttttgtcgctccagctcctgctgtagcttcttttcttgcatttcctttgccagcctctcctgctccctcttcttccgctcgcggagcgcctgctgaatcccccgatcgaatgtgagtttctcctcctcagtcagggcatcatattcttcctcatccatgttttggagaccctccttctctttctcaagagctcccttgtgcttgcgttcttcttgctcctttttggctttctcccgggccttcatggctgcgtaatcctgggccatgttgagaatgtatatatgctcccggctgccaatggccttcagcaggcagaggagggcggctgcagcattccgagcaaagagagtgtcgaggccatcaaacaccactcctcggtagcagtcactcagcagcctcctctccttccttcatggactgctctatggcagccctgatgcagagctcacaggcccggatccctgggatgttgttgctgttggccacagcttccagcacaatggagtcgatgctcaggcaggctgcgttgtagtacttggccacgctaacggcattggctgactttcctgacaagggtgtcccgtgaatgataatggcgatgcctttccggttcttggccaggcggccttctgcagaaatgtcaatgcccaggtggcgagcgattgctttgctcactgggttgttttccacctctccaacttcctccatggagtggctgtcaatgctctgaagcttgtcagtttggaaaatgattttttccaggctttcctcatcctcctcttcctctaggtaggttttggactcgaccaacagggcgtgccattcttccaggttggatgtgacagagatccctcggctcagcgatgtcctctttgtgctattggaggttccctgatctgatgaggttatatcttcctcttcattctcctgtgccagattctccagatatttcgccctcatctgctcctcttttgacttctttatctctttgaagtactcgtacagttctgggggcagcttctccccagggttgcggggaggcagcagcagggtgttgtaggaatcatagcccttcagcttccgcaagatcttttcttctatgagatactgctgatcaaattctaaggaataaaactcaatggggaagttgcagggattcttcactatcacctcggcctcgtctccaggtgcacaaagtagcagtggccccagatccaggactgaaggactaaattccaggcgtggctctagaccttgcccacgtgccaggagggtaagcttttgagcactctgggcaatctgaaacaccagggtttggctgtagaatttctcttcttttggcatgaatttcacttgcacgttggacttctcaccaggatccaagactccagaaatgggctggatttcgaagatccgtgtctttggctttaattcagcgcgtagtttctgtcttaagtacttcggcatgtgtttctccagcttgtcaacaggcttttggctctggacgaaccattcacaagggacttggagatgattggaaagctgaatagtttccaccaggcactgtccacactgaattgtggcaaagtccacttttccacgagagagagtcatggttggaatggtcaccttggcttggagacagatgtgaactgttggccctccaaccaccttgatgggcagaatgacttctttgcttccaacaggaagattggccccctgtgggtcaaatctcacttcaaatatttccgtttcacaatgaggcagattctttacacgatctagctcagtactgaatcctgtctcatgaaggacacgcttgtctgcatggaatgacactggaaagtgactggtgttgatgatcttgatgatgtgggttcggacttcgccaaggatgatgtagccaaagtccaggatgtactctggtagctggattttggccagtttgcggcgactccgatggctgaagcaggggtcatccataggatcaggggtggttgttttctgatgttctaggacatagctttggactataagtctttctacctccatctggagatgagcacttacctcagcaggctcgtcttctggcacttcctcagttattacgtcaaagtgatcgagcatttcacatttgttatactctttgtctgtgtttttcctggcttgattcaagaacatttcatacttttcatttgctgtgaggttcctggggagatcgaggcagatttggggaaagattccctctccgctcagagtgatattttctgggtccaggtgggcgatctgtatctggaaactccttttaaagacctcaggtactccaggtaggtagtaaacttttaatacctgctcttgatgtgaactgataaagccagacacaggcaggattagtggcactccagggagaaggttgtctggagaagactggtggtcagtcagaaccttgaactcaaagccaactttccccatgttcgtcagcgtgatttccctctctgtgacatggtcaaacagctgtaatccgtagtgaatatccttggtgtcaaaggaatagttgaccagggacgcctctcccttcagtgttatttcgtaggtgggtccttcttccacttcacacagagctttagcttgtgcaatgatgttagcgtgtccatagaaggtgaacgatatttggtggctactgtgtggctgcaacactccaaacaggggcaaaatatcaaacacttcttctatcccaatggaaagcatctcattctgttcacaggtctgtagggattcctgatcctccacctggctctggcttgagtatattctttctatttcagtagagctaatttttatttcttaacaaaatcatttaaatccatctcgggggactctactgtaactaggattgctggtgggctggcagcctctgaggttgctgggatggactccatctgggacagtggggcactgtagggcttctttggcaatgtcacaaaccttatctgattttcctcatcattcaccaagaagaaccagcgaaacttcacaaccaacggactgcagttggtgatggtaacgtagcgaatgagctcagtatcgttcaggatgcagccaaaatccagctcctttgtctcaaagctgaggttggggtaatgcacttctccgcgcaggtccaggctgtctatctgagggtgttccacatacttaattgctagaatttcttctgccacccagttgttcagatcgtttctgtaggaagggtcaaacttgatcagcaggtttttttcttcatcaatttccagtttaataggctcaggagttgccggcagcagggatttatcagtctcacatataaagaagggtccagatgttgacagcaacaagttcacgggcagggtggaaatgttctttacggccaagggctggtaatcaggtttcaggatactgttaggtttcctgggagtagcagaatagccttcgagtatcacatcaattgcctggcctgggtacagctccatgctggcggggtggagatgaaacacggggctctgtggatccctgggctcctgagagccactgggctggggttggacatgagcatgtcccttcttaacccggcccttcttactcagcttggcctggggtcggaagctatcattcatccagaacaactgttggatccgacgtcccttgttgatcaacttaaagtggtaatagtgggtatccaggctaaaatgtgcccccaaattgagttctggagcaaagggcttatctgaaacaatagtggaaccagttccggaagcctgaacaggaatccgataggtactgctattttcaatgtccaaaataacacagtccttgaatgtcagtgtgtcattcaggttggcggtcagtgccagttgaacatcagtttctggaggaaccatgccttcattgggttcaatcgtccaaagggattttttgtgtgccatgtgtgcctggaaaaatgcgggaatgaaggactggttgcataggttgagaatcctggaagagtcttttaggacgtagatattcccgaagtccacttgattgggatggacgtagataactgggccttctccagcgctctttaagtgacataccaaaggggggtcctggctcccaaagattgagatgtaaaccgtggatctgtgttctccagtgacctgggtctccaggaccagtggtatgtggatggtgctgcttggggagatgaccccgctgggggtggggctggaaaacagcacagtaggcacctcctcacacacctgaggctggacctcatagaatcctgggaggtcatcttgatcggcaagctggagtgttttctcatacgggtacttcaggaagcagtgcccaaagtccacctctgtattgaccaggtggagggcaggtacaacacaccttgctgcaattaagagcgccagcacctcttctccgatgccctccacgtccaccacgagtgccagctcgtatttctgtacagtgttggagcataatgtcaccctgatagcagcaaatccctgggggcgaatggtgccacagtcaggagagatggtgaattcttttggtttcattgaggatatttcttccttggtccaagacggtcttttgtagtccacatgctgctcacaatatgaaatgcttttatggccaaggccatccccagggatacgcagtttgtaagtcatggggatcaaagaggtattattgagggaacatatcaaggtatgaggaaacccaaaggaaacatcaccaaagtgcagagctggaacattaaaatggaaggtaggtccaatgacacagcctctaatggtcagtttcacaggctcaggtgacccattgacattgaccaggaactcttcttcaaagtttcccaggatggtagagctgaaggagatctggatagcttggactccacttggttcaatgatgccttccttgggactgaaaacaaagcaggcccccaaagctgaagttggaggggtcatgttgaagagagcatcgatgctgtctttgttgtacagtatcgcctcataacaatgtgcagatccagtgaaaactttcccaatatccagcaattcaaagttgaagtgaatcttaggtcccatgccttcccctttgattcggaggggcagacggatttctcggcctaaaatgtcgcagtaaatggtctgttgatagagcttggcttctagtgggttaaagtacacggtgatttcagctgatgagttgggccagacatcaccttccaggggctccacagtgaaaacgttattgaagaacagtttgctgtctccctgcaccagcctcctttgattcgcaaaggttcgggacagaacagaaagatgttctcggagtaaaggatcagtaatgcactcttcaaaaaactcatcagtctcatccttctcctctttgatcagatcatcacaggccctatatttttctctgtcctcttcttgctgggtagcaaataccttccacaggaaatgggcaatgatattactgcgattgtgaatggttatagttcgctgattggccagagatatgtaggttttctcgatggtcaaggaattcttatccagccttatattcatgtctatggcagctccatagagagatacaaacaccttttcacctgtgtcataacacacgataagtcttccactgtgatcgcccacactctgtggctcaaactccacttccagttgcatggactctcccacattaagagttccaatagctggttctatagagaaaggcctacaagttttgatgtgaaatacagcatttttgttgccaatgtttcgtaccagcagaatcttctgggtgctgtatttgacaggacaagtggaaaaattcagcttgtcaggaaaatcgagaatggctcgtgcccctctagctttgatgggtacaataaacttttctctttcagtaacacaggtcaacgtatgggcgtaatcagtgacatcagcaacatgatggattccatcgccagcagcctggactccaggaggcaccccaggcgtggccgatgtgcacaggtaggagcatgtcctctgcgtggcctctgcactggaagagcttcaaggccttttcctccagggctgaggggatttgtgtttcgcctctgtttgtttttgtgtacttctgtttggcgaaactttcaagcacgcagagcaacgttctgatagatagtgcagagaggagctgcgcagcatcctggagccgaaagttacaaggaagagaccaaaaccggtaaagtcacggatgttgtggcccgaacctaagcatggtggtgtatgccagtagtccagaaattcaagattacagtgtgctatggcaccactacactccgtcctgagcaacagacaaagaccttgtctctgctgtgtctccagatcatgtgcatggctgcatgcagtctagggttctccaccaacaggcagatccacaatgccctgctacaatccagatttccaaaaccctttagactgcattaatagaaacataatacctgtagtcccaattactcaggaggcagaggtggaaggattgcttgagcccaggtgtttgaggctgcagtgagctataattgtgccattgcactccagcctgggtgacagaatgagacgttgtccaaagtgtcaaagttggtaaatggcagagctggaattcaaagagtctgattccaaagtctatatagtccggcgtgatcattaaaggaattccttgtgttcaaagagcagtgcttgaaaaccaagctcatttgtgcctgcagaaatgccagcctctggggtagaagaaatgtcatactttgatcatcttccacactgctctgggcatactccgtcacaaactacgttgtgtgaatctgaggactgctttagaaatgagttcccaaattgctcaagaaatagttcaggctgtaattctgaaaagccttctgctcactcaggtccagtgatcacctctgaggagtgagattagagcagcgaagagacttccaattcttactttatacacttctgtattgtttgaaccgctctaatcgctccgattttccaaggccttgctcagtagtcctgccaggcgggccctgaggctggaagggatgggggagttcggtgagtgcgccctgcctacagcgcccagtggaatcgctagtacctgtctctgtggcgcaatcggtcagagcgttcggctattaaccgaacggtgagtagttcaagaccacccagggacgcctgttctagcttttaaagcattcatgtattatcatcactagagaatctccccctattcttcccatagtcctaagtccgaaaggttggttccaggccagccagggatatgcccatttcaggaaggtttttctcttctcaggattctagtcacagttaacagggatccctatcaagagccaccccactcagagatccaattctgacagagcatctcctgaaatgtcaggttgtcttgtgcc

SEQ ID NO: 15885 - RNA, 276 nt, Homo sapiens
  source 1..276: mol_type = other RNA
gctgggattacaggcatgagccatcacacccgcccctcattttaatttgattacctctgtaaatacctctgtctccaaatgagatttcatcctgagcagctgggggttaggacttcaatatatgaatttgacagggagggtagaaggagagaacagaattcaacccacagcagcaacaatctaatagcttcctgtgagcaagcaaagagaatgttcattgtcagtctcataggcgccattccctattcatacgttacttgtgctctctcatattcc

SEQ ID NO: 15886 - RNA, 4794 nt, Homo sapiens
  source 1..4794: mol_type = other RNA
gctgggattacaggcatgagccatcacacccggccttccaagtgcctttctgatgcctcagccacaccagcacctccctgggacctccctgtgatctgccaactaaaggggtagcacctggcagaggtggggtgttcctgcactctagccagcatgatacgctgtcccgatggttaagtattttggttgtcatctctgctgtatccttctcagcttccatcaaccctttgttggctgacttcacctgtcctgaaatattcagctgtagtctcctctccctaccacacccacttccctctgaaaactcaccaggctgggccgacagcacctggcagtgcggataagggcatggcctgccctctgcggtgtcagaactccattcagaaggcccctccccaggtggatgtggttccaggggctggcgaggagtcaggcacaaccacactggctgtgaatttgagtaacaggggcctggggtttctggtagcagcctcttgtccaggcctggaggtccacagatcaaggggtgtgcctctggggaccaaggatatgccacactgggggtgtaatggggaaaaatctggcaagctgggtgcacagttgcatcctggggccgagagccaggggtgggctcggagggacccccccgccttttcctctgtgggtgtcgggcagagaggctggatttttgcaagttgaacagactgctggtactggggcagatgctggaggcgtcaactgggccaggggctggctcagggagggccctggggcactgtgggttagagagccgccccgaaggggctgctgagttggatctggtgacttgctgatcaggagaaggtggctctggctggggctgtgtccgaggaataggaggcctggactgggggactccggtttctgggccaggcttcctgccatgccactggaaccgctttttgtagtggtggtgccggtggcggtggtagtggacatggctggaaacctgggtttcccctgtgggcaccaccgagtccaaggaacgaggccgagaggtcacactaggctgcatgtccactcgctggggatcccctttagggctgcagtacactagggggtcaaagtcactgcttagggagctgcagaaagtagaactgctgccatggaccccctgtaggctgatgtccgtgcagttgaccacagagtcactggaagagccatgacagggccctgagctggagtcactggctggcccatctgccaggtacccactgcgttctgtgcaatagctttctccagatccactgctgtcagggggcctggcccggcgtaggggcactgggcaagcagcagggtgctgtgaggtggattggaggtggctcagtccccagccttgtgcataggggtgctgggctcctgccaggcgctgctgctctcctggagcccggggatgtgcagctctggggaagcggtgatgccgagggcccatgcctggctcctgggatggcaggaagggaccaggtcgtgggggccgagccactgcactccgggaagggcccaacaggtaggcagcagggaggtggtagtgggcatggccgggatgctggcgaatgaggtggagtcttcgacctggttcttggtaagatcgagagggtcccagggactgggaaaatgaatctccctctgtgatgttgaacatgcagagggggcaagtccgatgctgatgtaaccaggggtccacacagttacgatggaactcatggaggcaggaaatgacccgtagctcctgcccctcagagaactcctccagacagatggcacacacaggggctgagctgcagctgctccctgagtctggccactcaccccgggcctgcctgcagctggcctggtacctcctggtggccagctggctgatggcccaggctgttctctgctgaagcggatccggcctgctgtggcgggggcggcaccggatgcgcagcaccgaagccaggatgatcacaaagatggtgcccaccactgtcattaggatccacacatcataatctggccaggccgggggctccttcagctcaatcctcacatgggccttttggttcttgtacacaaactccatcagcttctcagcgtcattaccccagatcaacaccactggccaggtcagccccagcggctgctgcagctgctcagcagcagctcgatcctcagtgatgtcaaagaggacagcactggctcctcgctcacccgccatccgagccttgctagccagtgacaggcaggggcggggggcccgtcgaggactctccagcttgacgatgctgatgaatccaggctccagattgtcgtcatcactggcattgcacaggtacagcgggtgggactgcattaattttccttctgctggagttatttcagcaacaccagcaaacacaccttccaaagtgagattcagttttcctgtggggtccattttcaaggggatcactctgataatagctttctgttctgctgatctttcagactccaccgctgctgccagtaccagtcctgtgcgtccaaagcctgcctgcagggtagccatcagcagccagggccagagggcagccagctgcagctggtggccaccactcatgctaccagctgcagcaatgcacttcaaccatacatactgcttccactagctaataccaaatgcaggttctcagatccagacaaatggaggaaaagaacatttatgcttccgtttcagaaagccaagtcgtagttttggcccttcctttctctaaagtttattcccaaaaacaggtagcattcctgattgggcagagaagaggatattttcagcccacatctgctgcaggtatgtcattttctcccatcttcactgtgactagtaaagatctcaccacttctctttggaatttccaactttgcttgtgattgaatgtcacttcgtgaatttgtattatgtcagatcacttggcattgctcttccatatgcatcaagttgccaggcactgttgcgctgtcgggcccactggaatccacgggggtgaaacaaattcaattatgcttttacagatcctgctcaaaaaaggtttcaactgcttaaccaagtacagctcattcttccaccttcttactctgcaaccaaaccaagtgccccatactacaggtaggtgccgagaaattccgcagcagaaaatccaaaatcatttctgaaacctccttgctaacaaaagttctttttttctccaaacagcatataaaatgatcaagtcttgaaagagaaaagaagcaaagtagcaaatacatcaacaattcactatcagaaacacataaaatcccagagagagagaaggcagtatctctgaatcatggatggacttggaaagttcggaaggattccgagtgcttcctttcagaaagacaattctggatcaactccctagagcaggaagcctgtggtttgtaattggtgttctagctctgactccctcccctgggactgcaatcacgctctctacctgctgacaaagtgagggtggagctgctagaggcaaccactccccaccctgcccccctcctcctggtgctcacacacaacacttacttaaccagacccgttctttcgctctcccccctccctcagctcctctactccctctactgagccacagctaaactgcatccaattcgatcccgagtacctttctctgggtaagcaagctaccacatgcaaatcagggccactcaaagatatctaagcagactctgcacccaacagagcatagatgatggtatgaggaaataaacagaaaaaaataaaggtaatccggaagataaaagaatggacacaaggttttgcaaatataagttcaaaaggatttctgctcattccaagtttgagtgtctataaatggcagaaagccagaataaagtgatcctgtgttttagtacttactgatttattgctgcttatgtctgctaccctgggaagggctctgtccattttatgcttagcttttcttcagctcttactaatttaaattcagtagctctgtctaaactgtgcctatatggaactttcaaatcaggttgatgtcagatgtctggaatccaactgttattttcttttcaatctttgggaggtgaaataatactatggatcagacctatgccttcaatgtaagactccaaataagtccatgtcataaatacaagccaaagggtaaaatatgattaatgagaagaacataggcaaaaagaaaatgaatttctggctaattaccacattcatgaactataatccttattactaccctgccattagaaataatacaacagtttctaatacatttataacatttgaagtttcaaattaccagattatatttgactgtggtgagacattttatttctgaaccgctgccataaactttcaaaattatacaaatgaacaacaatgtggatatagttaaatctagtgaactgtacacttaaaaatggttatgatagtaaattttatgtgtttcttacctcatgtaaaaacgaatctctgatcatctgtaaaatgctgatgataataattacgataggtctgttgtaaagattaaatgacataatgcctctgaaagcaaaaaggatgagtagcctattgaccttcaacattgtttcccctgtagataaggtttatgacagtagtttcagaatttcagatctaataactaacctagatcaaagacaaattcgaaaataaattttttgtttatttttgttgtttgagacagggtcttgtgttacccacgc

SEQ ID NO: 15887 - RNA, 3517 nt, Homo sapiens
  source 1..3517: mol_type = other RNA
gctgggattacaggcatgagccatcacacccggccttccaagtgcctttctgatgcctcagccacaccagcacctccctgggacctccctgtgatctgccaactaaaggggtagcacctggcagaggtggggtgttcctgcactctagccagcatgatacgctgtcccgatggttaagtattttggttgtcatctctgctgtatccttctcagcttccatcaaccctttgttggctgacttcacctgtcctgaaatattcagctgtagtctcctctccctaccacacccacttccctctgaaaactcaccaggctgggccgacagcacctggcagtgcggataagggcatggcctgccctctgcggtgtcagaactccattcagaaggcccctccccaggtggatgtggttccaggggctggcgaggagtcaggcacaaccacactggctgtgaatttgagtaacaggggcctggggtttctggtagcagcctcttgtccaggcctggaggtccacagatcaaggggtgtgcctctggggaccaaggatatgccacactgggggtgtaatggggaaaaatctggcaagctgggtgcacagttgcatcctggggccgagagccaggggtgggctcggagggacccccccgccttttcctctgtgggtgtcgggcagagaggctggatttttgcaagttgaacagactgctggtactggggcagatgctggaggcgtcaactgggccaggggctggctcagggagggccctggggcactgtgggttagagagccgccccgaaggggctgctgagttggatctggtgacttgctgatcaggagaaggtggctctggctggggctgtgtccgaggaataggaggcctggactgggggactccggtttctgggccaggcttcctgccatgccactggaaccgctttttgtagtggtggtgccggtggcggtggtagtggacatggctggaaacctgggtttcccctgtgggcaccaccgagtccaaggaacgaggccgagaggtcacactaggctgcatgtccactcgctggggatcccctttagggctgcagtacactagggggtcaaagtcactgcttagggagctgcagaaagtagaactgctgccatggaccccctgtaggctgatgtccgtgcagttgaccacagagtcactggaagagccatgacagggccctgagctggagtcactggctggcccatctgccaggtacccactgcgttctgtgcaatagctttctccagatccactgctgtcagggggcctggcccggcgtaggggcactgggcaagcagcagggtgctgtgaggtggattggaggtggctcagtccccagccttgtgcataggggtgctgggctcctgccaggcgctgctgctctcctggagcccggggatgtgcagctctggggaagcggtgatgccgagggcccatgcctggctcctgggatggcaggaagggaccaggtcgtgggggccgagccactgcactccgggaagggcccaacaggtaggcagcagggaggtggtagtgggcatggccgggatgctggcgaatgaggtggagtcttcgacctggttcttggtaagatcgagagggtcccagggactgggaaaatgaatctccctctgtgatgttgaacatgcagagggggcaagtccgatgctgatgtaaccaggggtccacacagttacgatggaactcatggaggcaggaaatgacccgtagctcctgcccctcagagaactcctccagacagatggcacacacaggggctgagctgcagctgctccctgagtctggccactcaccccgggcctgcctgcagctggcctggtacctcctggtggccagctggctgatggcccaggctgttctctgctgaagcggatccggcctgctgtggcgggggcggcaccggatgcgcagcaccgaagccaggatgatcacaaagatggtgcccaccactgtcattaggatccacacatcataatctggccaggccgggggctccttcagctcaatcctcacatgggccttttggttcttgtacacaaactccatcagcttctcagcgtcattaccccagatcaacaccactggccaggtcagccccagcggctgctgcagctgctcagcagcagctcgatcctcagtgatgtcaaagaggacagcactggctcctcgctcacccgccatccgagccttgctagccagtgacaggcaggggcggggggcccgtcgaggactctccagcttgacgatgctgatgaatccaggctccagattgtcgtcatcactggcattgcacaggtacagcgggtgggactgcattaattttccttctgctggagttatttcagcaacaccagcaaacacaccttccaaagtgagattcagttttcctgtggggtccattttcaaggggatcactctgataatagctttctgttctgctgatctttcagactccaccgctgctgccagtaccagtcctgtgcgtccaaagcctgcctgcagggtagccatcagcagccagggccagagggcagccagctgcagctggtggccaccactcatgctaccagctgcagcaatgcacttcaaccatacatactgcttccactagctaataccaaatgcaggttctcagatccagacaaatggaggaaaagaacatttatgcttccgtttcagaaagccaagtcgtagttttggcccttcctttctctaaagtttattcccaaaaacaggtagcattcctgattgggcagagaagaggatattttcagcccacatctgctgcaggtatgtcattttctcccatcttcactgtgactagtaaagatctcaccacttctctttggaatttccaactttgcttgtgattgaatgtcacttcgtgaatttgtattatgtcagatcacttggcattgctcttccatatgcatcaagttgccaggcactgttgcgctgtcgggcccactggaatccacgggggtgaaacaaattcaattatgcttttacagatcctgctcaaaaaaggtttcaactgcttaaccaagtacagctcattcttccaccttcttactctgcaaccaaaccaagtgccccatactacaggtaggtgccgagaaattccgcagcctgaaaaaataatccatgcaggtcaaaggcagaaatttactccgggatgagagatgctgtcccctagaactaaattaaacacttacagaaaatccaaaatcatttctgaaacctccttgctaacaaaagttctttttttctccaaacagcatataaaatgatcaagtcttgaaagagaaaagaagcaaagtagcaaatacatcaacaattcactatcagaaacacataaaatcccagagagagagaaggcagtatctctgaatcatggatggacttggaaagttcggaaggattccgagtgcttcctttcagaaagacaattctggatcaact

SEQ ID NO: 15888 - RNA, 2880 nt, Homo sapiens
  source 1..2880: mol_type = other RNA
gctgggattacaggcatgagccatcacacccggccttccaagtgcctttctgatgcctcagccacaccagcacctccctgggacctccctgtgatctgccaactaaaggggtagcacctggcagaggtggggtgttcctgcactctagccagcatgatacgctgtcccgatggttaagtattttggttgtcatctctgctgtatccttctcagcttccatcaaccctttgttggctgacttcacctgtcctgaaatattcagctgtagtctcctctccctaccacacccacttccctctgaaaactcaccaggctgggccgacagcacctggcagtgcggataagggcatggcctgccctctgcggtgtcagaactccattcagaaggcccctccccaggtggatgtggttccaggggctggcgaggagtcaggcacaaccacactggctgtgaatttgagtaacaggggcctggggtttctggtagcagcctcttgtccaggcctggaggtccacagatcaaggggtgtgcctctggggaccaaggatatgccacactgggggtgtaatggggaaaaatctggcaagctgggtgcacagttgcatcctggggccgagagccaggggtgggctcggagggacccccccgccttttcctctgtgggtgtcgggcagagaggctggatttttgcaagttgaacagactgctggtactggggcagatgctggaggcgtcaactgggccaggggctggctcagggagggccctggggcactgtgggttagagagccgccccgaaggggctgctgagttggatctggtgacttgctgatcaggagaaggtggctctggctggggctgtgtccgaggaataggaggcctggactgggggactccggtttctgggccaggcttcctgccatgccactggaaccgctttttgtagtggtggtgccggtggcggtggtagtggacatggctggaaacctgggtttcccctgtgggcaccaccgagtccaaggaacgaggccgagaggtcacactaggctgcatgtccactcgctggggatcccctttagggctgcagtacactagggggtcaaagtcactgcttagggagctgcagaaagtagaactgctgccatggaccccctgtaggctgatgtccgtgcagttgaccacagagtcactggaagagccatgacagggccctgagctggagtcactggctggcccatctgccaggtacccactgcgttctgtgcaatagctttctccagatccactgctgtcagggggcctggcccggcgtaggggcactgggcaagcagcagggtgctgtgaggtggattggaggtggctcagtccccagccttgtgcataggggtgctgggctcctgccaggcgctgctgctctcctggagcccggggatgtgcagctctggggaagcggtgatgccgagggcccatgcctggctcctgggatggcaggaagggaccaggtcgtgggggccgagccactgcactccgggaagggcccaacaggtaggcagcagggaggtggtagtgggcatggccgggatgctggcgaatgaggtggagtcttcgacctggttcttggtaagatcgagagggtcccagggactgggaaaatgaatctccctctgtgatgttgaacatgcagagggggcaagtccgatgctgatgtaaccaggggtccacacagttacgatggaactcatggaggcaggaaatgacccgtagctcctgcccctcagagaactcctccagacagatggcacacacaggggctgagctgcagctgctccctgagtctggccactcaccccgggcctgcctgcagctggcctggtacctcctggtggccagctggctgatggcccaggctgttctctgctgaagcggatccggcctgctgtggcgggggcggcaccggatgcgcagcaccgaagccaggatgatcacaaagatggtgcccaccactgtcattaggatccacacatcataatctggccaggccgggggctccttcagctcaatcctcacatgggccttttggttcttgtacacaaactccatcagcttctcagcgtcattaccccagatcaacaccactggccaggtcagccccagcggctgctgcagctgctcagcagcagctcgatcctcagtgatgtcaaagaggacagcactggctcctcgctcacccgccatccgagccttgctagccagtgacaggcaggggcggggggcccgtcgaggactctccagcttgacgatgctgatgaatccaggctccagattgtcgtcatcactggcattgcacaggtacagcgggtgggactgttgcgctgtcgggcccactggaatccacgggggtgaaacaaattcaattatgcttttacagatcctgctcaaaaaaggtttcaactgcttaaccaagtacagctcattcttccaccttcttactctgcaaccaaaccaagtgccccatactacaggtaggtgccgagaaattccgcagcctgaaaaaataatccatgcaggtcaaaggcagaaatttactccgggatgagagatgctgtcccctagaactaaattaaacacttacagaaaatccaaaatcatttctgaaacctccttgctaacaaaagttctttttttctccaaacagcatataaaatgatcaagtcttgaaagagaaaagaagcaaagtagcaaatacatcaacaattcactatcagaaacacataaaatcccagagagagagaaggcagtatctctgaatcatggatggacttggaaagttcggaaggattccgagtgcttcctttcagaaagacaattctggatcaact

SEQ ID NO: 15889 - RNA, 2913 nt, Homo sapiens
  source 1..2913: mol_type = other RNA
gctgggattacaggcatgagccatcacacctatttattttttgtagagatatggtcttgctgtgttgcccaggctggtcttgaactaatgggctcaaccaatcctcctggcttggccccccaaaatgttgggattacaggcctgagccaccgcactcggacttttttatttttgagacagggtttcactctgtcacccaggctggagtgcagtgacacgatcatagctcactgcagactcgaactcctgggctcaagaaatcttctgcctcagactcccgagtagttgagactacaggtatgtgccaccacacccggctgatttttgcattttttgtagagatgaggtctatgttgcccaggctggtcttgaatttctggcctcaagcgatcctccttcctcagcctcccaaagtgcaggggttacaggtgtgaggcactgcaccagccccacattacaaagcttttagagccaggccaggaaggttcaaggttgtagtacaacatgatcatgcttgtgaaaagccactgcagtccagcctggacaacacagcaagacctgcttctcttaaaaacaaacaaacaaaaaacacctcttggctgggcatggtggctcatgcttgtaatcccagcactttgggaggctgaagcaggtggatcacttgaggtcaggagttcaagaacagcctggccaacatggtgaaaccctatctctactaaaaatacaaaaattagctgggctttacataaaaccgggcagggcatggtggctcacatctgtaatcacagctcagtctcctggggactacatgcctgtagtcgcagctactcaggaggctgaggcaggagaattgcttaaacccagaggtggaggttgcagtgagctgagatcacaccactgcactccagcttgggtgacagagcaagactccgtcttaaaaaacaaaacaaaaaaacaaacaaaaaaacacctcttaaaaagttaattttactaagccttttaaaggaataagacagccttcagaagtcaggcactgtggctcatctgtaatcccagcgttctgggaggctgaggcaggcagatcacctgaggtcaggagtttgagacagcctggccaacatggtgaaaccctgtctctactaaaaatacaaaaattagccaggtgtggtggtgcatgcctgtagtcccagctcggaggctgaggcaggagaatcgcttgaaccccggaagtggaggttgcagtgagccgagaatgtgccaggtgacacagctagactagactccgtctcaaaaaaaaaaaaatagctttcagaaaacagcgttactcaaaatgccttgtgtttaaattttaaaactttattggctgacggaaaactgccatactttcttcccactaccatcctgctattcctgaattcaatttgcaaaagaagcatagaccaagaagggttccttaggtgctcaacagaatttaaagtgcgacagatatgtttacaattagaaaataaaacttctctctcagtttaaagaaatttttttctttgtacatattttaaagtacagttgtgttttctttttaggaactgtggaaaatgcctatttataatgtctttggaaggataccccattttgtaattgtggtcttccagattcttctgggttaacatgttgagatgtattccacggtactcgcatttctgataaatccatattgtctcgaagagacttcctttcagctttctgacatcttatcaagaattagtagaggggcaagaattcttgccctgttagtttccacaatgcagccatttaacaccatctcatccaaaatgatgtgtactttatccaaattaaacattatatctaattcactcactcggctgaaatactcatctaaaacttccacaaagttatgaatgaattcataaatagccatctcgttctcagtgtcattaactccaaccacaatgaagagagctgcatactgccgatatatcagcttaaaatccttatattcaatgaaagagcattgttcattggatcgagagagacagctctttatgacttctgtttccagaagtgtacgcttattaatatccacatgttcatagtacttagaaagtcgagtctgcccttgtttattcaccatgaggaaaaattttatcatttttctttcctggccagtatttttccaaatacagttcaaaagttatgacaagggatggctgtaactggaacagtgcttttattttctgtttcgatcaaaatagtctattgatgacaatatttgtgagcccattcatttctaccgtatcaaattgttagtctagccagtctccttcaaacttctctccctctacccatcatcgtcaagatctaaaggaattcactacctcttcttctcccaagaaaaaaaaaatcgctcctccccctctcccaacccccccacaacccattccagaaaaggaaagaagaggggacgcaaagtggaataagttacgacgggcgaccgagcgcatagaaatgggaccaaagcccaggctcaagacagagacgaggaatcagtaaccacagccggaggatcttggctatttgccagcagagaactgactggttctaagaaaccagaggcagagcgagtgacaggaagggaaagagggcccacccttgggactgcctgaaacactcaaagaatgaaaaagaaacgtcaggaatccgagacgggatgcggtcggccagagcgaccagccaggttaacaaccagctcagaaagccgggacacgggtgagagacccctgggaaggaaacagcgcccggggacggcctgctaaaaggaaactgataaccaggaagcctaaggccgcctcgcttccaaaagtcagagtcggagcccaggtgtccggtagctgcggc

SEQ ID NO: 15890 - RNA, 2431 nt, Homo sapiens
  source 1..2431: mol_type = other RNA
gctgggattacaggcatgagccatcacacctatttattttttgtagagatatggtcttgctgtgttgcccaggctggtcttgaactaatgggctcaaccaatcctcctggcttggccccccaaaatgttgggattacaggcctgagccaccgcactcggacttttttatttttgagacagggtttcactctgtcacccaggctggagtgcagtgacacgatcatagctcactgcagactcgaactcctgggctcaagaaatcttctgcctcagactcccgagtagttgagactacaggtatgtgccaccacacccggctgatttttgcattttttgtagagatgaggtctatgttgcccaggctggtcttgaatttctggcctcaagcgatcctccttcctcagcctcccaaagtgcaggggttacaggtgtgaggcactgcaccagccccacattacaaagcttttagagccaggccaggaaggttcaaggttgtagtacaacatgatcatgcttgtgaaaagccactgcagtccagcctggacaacacagcaagacctgcttctcttaaaaacaaacaaacaaaaaacacctcttggctgggcatggtggctcatgcttgtaatcccagcactttgggaggctgaagcaggtggatcacttgaggtcaggagttcaagaacagcctggccaacatggtgaaaccctatctctactaaaaatacaaaaattagctgggctttacataaaaccgggcagggcatggtggctcacatctgtaatcacagctcagtctcctggggactacatgcctgtagtcgcagctactcaggaggctgaggcaggagaattgcttaaacccagaggtggaggttgcagtgagctgagatcacaccactgcactccagcttgggtgacagagcaagactccgtcttaaaaaacaaaacaaaaaaacaaacaaaaaaacacctcttaaaaagttaattttactaagccttttaaaggaataagacagccttcagaagtcaggcactgtggctcatctgtaatcccagcgttctgggaggctgaggcaggcagatcacctgaggtcaggagtttgagacagcctggccaacatggtgaaaccctgtctctactaaaaatacaaaaattagccaggtgtggtggtgcatgcctgtagtcccagctcggaggctgaggcaggagaatcgcttgaaccccggaagtggaggttgcagtgagccgagaatgtgccaggtgacacagctagactagactccgtctcaaaaaaaaaaaaatagctttcagaaaacagcgttactcaaaatgccttgtgtttaaattttaaaactttattggctgacggaaaactgccatactttcttcccactaccatcctgctattcctgaattcaatttgcaaaagaagcatagaccaagaagggttccttaggtgctcaacagaatttaaagtgcgacagatatgtttacaattagaaaataaaacttctctctcagtttaaagaaatttttttctttgtacatattttaaagtacagttgtgttttctttttaggaactgtggaaaatgcctatttataatgtctttggaaggataccccattttgtaattgtggtcttccagattcttctgggttaacatgttgagatgtattccacggtactcgcatttctgataaatccatattgtctcgaagagacttcctttcagctttctgacatcttatcaagaattagtagaggggcaagaattcttgccctgttagtttccacaatgcagccatttaacaccatctcatccaaaatgatgtgtactttatccaaattaaacattatatctaattcactcactcggctgaaatactcatctaaaacttccacaaagttatgaatgaattcataaatagccatctcgttctcagtgtcattaactccaaccacaatgaagagagctgcatactgccgatatatcagcttaaaatccttatattcaatgaaagagcattgttcattggatcgagagagacagctctttatgacttctgtttccagaagtgtacgcttattaatatccacatgttcatagtacttagaaagtcgagtctgcccttgtttattcaccatgaggaaaaattttatcatttttctttcctggccagtatttttccaaatacagttcaaaagttatgacaagggatggctgtaactggaacctgagatgctgccttactcacttggattctctgtagttattccttacttagtgactcatcaacgctttcagcactgaatttttctttttacagtactctccactagatctcctttcccccatccgtttctttatctataaaaaaaccaaaccagacgatcgatgctgtatttatgaaacgactgaagagattt

SEQ ID NO: 15891 - RNA, 2377 nt, Homo sapiens
  source 1..2377: mol_type = other RNA
gctgggattacaggcatgagccatcacacctatttattttttgtagagatatggtcttgctgtgttgcccaggctggtcttgaactaatgggctcaaccaatcctcctggcttggccccccaaaatgttgggattacaggcctgagccaccgcactcggacttttttatttttgagacagggtttcactctgtcacccaggctggagtgcagtgacacgatcatagctcactgcagactcgaactcctgggctcaagaaatcttctgcctcagactcccgagtagttgagactacaggtatgtgccaccacacccggctgatttttgcattttttgtagagatgaggtctatgttgcccaggctggtcttgaatttctggcctcaagcgatcctccttcctcagcctcccaaagtgcaggggttacaggtgtgaggcactgcaccagccccacattacaaagcttttagagccaggccaggaaggttcaaggttgtagtacaacatgatcatgcttgtgaaaagccactgcagtccagcctggacaacacagcaagacctgcttctcttaaaaacaaacaaacaaaaaacacctcttggctgggcatggtggctcatgcttgtaatcccagcactttgggaggctgaagcaggtggatcacttgaggtcaggagttcaagaacagcctggccaacatggtgaaaccctatctctactaaaaatacaaaaattagctgggctttacataaaaccgggcagggcatggtggctcacatctgtaatcacagctcagtctcctggggactacatgcctgtagtcgcagctactcaggaggctgaggcaggagaattgcttaaacccagaggtggaggttgcagtgagctgagatcacaccactgcactccagcttgggtgacagagcaagactccgtcttaaaaaacaaaacaaaaaaacaaacaaaaaaacacctcttaaaaagttaattttactaagccttttaaaggaataagacagccttcagaagtcaggcactgtggctcatctgtaatcccagcgttctgggaggctgaggcaggcagatcacctgaggtcaggagtttgagacagcctggccaacatggtgaaaccctgtctctactaaaaatacaaaaattagccaggtgtggtggtgcatgcctgtagtcccagctcggaggctgaggcaggagaatcgcttgaaccccggaagtggaggttgcagtgagccgagaatgtgccaggtgacacagctagactagactccgtctcaaaaaaaaaaaaatagctttcagaaaacagcgttactcaaaatgccttgtgtttaaattttaaaactttattggctgacggaaaactgccatactttcttcccactaccatcctgctattcctgaattcaatttgcaaaagaagcatagaccaagaagggttccttaggtgctcaacagaatttaaagtgcgacagatatgtttacaattagaaaataaaacttctctctcagtttaaagaaatttttttctttgtacatattttaaagtacagttgtgttttctttttaggaactgtggaaaatgcctatttataatgtctttggaaggataccccattttgtaattgtggtcttccagattcttctgggttaacatgttgagatgtattccacggtactcgcatttctgataaatccatattgtctcgaagagacttcctttcagctttctgacatcttatcaagaattagtagaggggcaagaattcttgccctgttagtttccacaatgcagccatttaacaccatctcatccaaaatgatgtgtactttatccaaattaaacattatatctaattcactcactcggctgaaatactcatctaaaacttccacaaagttatgaatgaattcataaatagccatctcgttctcagtgtcattaactccaaccacaatgaagagagctgcatactgccgatatatcagcttaaaatccttatattcaatgaaagagcattgttcattggatcgagagagacagctctttatgacttctgtttccagaagtgtacgcttattaatatccacatgttcatagtacttagaaagtcgagtctgcccttgtttattcaccatgaggaaaaattttatcatttttctttcctggccagtatttttccaaatacagttcaaaagttatgacaagggatggctgtaactggaacctgtgctgctcaggttgtgatggtcctctcaacggcttttcctggagtccccctccctctttcccgcataagcttgctccccaaccttcactggctacgcggtgcgggcctcctcggggcagccattttggcttttagt

SEQ ID NO: 15892 - RNA, 1603 nt, Homo sapiens
  source 1..1603: mol_type = other RNA
gctgggattacaggcatgagccatcacacctggccaatttttctaaaagtctgaaattaagtcaaaattttgaaaaagttatagcaattatggcaatctcaattatgggtaaatgtgtgtcacattatctcctttacattttaagtatttcataattaaaaaaaaaaagcagagaaaattgtttatcagaggaaacctcagaagagatgaggcagtcgtcagcaagtagaaggctccctttcaggaaactgaaaccgggtgccaggtggctgcagagcgggtgagagcttagcccccacctctccactggaacctagtgaccccatgcagataacaacctgcccaactcttcagccctgacctggcatcatatttatctataactggcagttcttctctgacaggatagattaataaacattaaaacacatctaaaatttatttacctgttgttcatgcaggtatgctagtgttcagtcagcatttgtaagacattcgttgtaaacaaagcactgaattagacagaatagatgaacagaaagataaacaagacctggccaaatgttgccccaaatccatacctgatggagacaggaagggcctttagtgcttgtgtgtcagtggtgatactattcactttcattttttttctgccacatttcattttcataccaattctggttagtgggtttcatttattctcattttacagatgagaacgaccagagatgttagcttgcccaaaattactcaaatactaaatgacaaagctaagagtatcatgtccgaggtaacaggtctgactccagagttcatgttctctccttatcatcctattttataagtcacaaaaacatgaatacagcaaaatttcacttactcaacactcccggggatgagtcatgctggacagatgaataagtgaaaggctatcctctgagaaatattgttcaaaaccttccaaggttagagaacagaagactccagaagcctttggacagtcttttcctccctgtgattcttttcctcttgggcttctgggatttcaaactcggtacatctggtctcttggagacacatcctccctggaagctccagcagaagatggccaaagaccccttttgccttttctgcttctccaaagcacaaatgagagactgataattcagaaataattctaatacctggctaattttcgtatttttagtaaagatggggtttcgccatgttggccaggctggtttcgaactcctgacctcaggtgatctgcctgccttggcctcccaaagtgctgggattacaggcatgagccaccgtgcccggcctttccagtggttttcgaagtgctcccgacagcctcccatgagggaaagtgtgggaatggggatagggggtgctggctggttgagataactctcattcttcctcatttcaactacgttaatctgttctacatactgaatttattggtaagctttgatctgaagggttccatacctttttcactgagagcctttccactcccctccccttctagtagtcgtgaacttcagaccctcgcttcgactcccactgccataactgtttttaaccaagcttccct

SEQ ID NO: 15893 - RNA, 1290 nt, Homo sapiens
  source 1..1290: mol_type = other RNA
gctgggattacaggcatgagccatcacacctggccaatttttctaaaagtctgaaattaagtcaaaattttgaaaaagttatagcaattatggcaatctcaattatgggtaaatgtgtgtcacattatctcctttacattttaagtatttcataattaaaaaaaaaaagcagagaaaattgtttatcagaggaaacctcagaagagatgaggcagtcgtcagcaagtagaaggctccctttcaggaaactgaaaccgggtgccaggtggctgcagagcgggtgagagcttagcccccacctctccactggaacctagtgaccccatgcagataacaacctgcccaactcttcagccctgacctggcatcatatttatctataactggcagttcttctctgacaggatagattaataaacattaaaacacatctaaaatttatttacctgttgttcatgcaggtatgctagtgttcagtcagcatttgtaagacattcgttgtaaacaaagcactgaattagacagaatagatgaacagaaagataaacaagacctggccaaatgttgccccaaatccatacctgatggagacaggaagggcctttagtgcttgtgtgtcagtggtgatactattcactttcattttttttctgccacatttcattttcataccaattctggttagtgggtttcatttattctcattttacagatgagaacgaccagagatgttagcttgcccaaaattactcaaatactaaatgacaaagctaagagtatcatgtccgaggtaacaggtctgactccagagttcatgttctctccttatcatcctattttataagtcacaaaaacatgaatacagcaaaatttcacttactcaacactcccggggatgagtcatgctggacagatgaataagtgaaaggctatcctctgagaaatattgttcaaaaccttccaaggttagagaacagaagactccagaagcctttggacagtcttttcctccctgtgattcttttcctcttgggcttctgggatttcaaactcggtacatctggtctcttggagacacatcctccctggaagctccagcagaagatggccaaagaccccttttgccttttctgcttctccaaagcacaaatgagagactgataattcagaaataattctaatacctttttcactgagagcctttccactcccctccccttctagtagtcgtgaacttcagaccctcgcttcgactcccactgccataactgtttttaaccaagcttccct

SEQ ID NO: 15894 - RNA, 1397 nt, Homo sapiens
  source 1..1397: mol_type = other RNA
gctgggattacaggcatgagccatcacacctggcccctagccttcttgactgatgccagatccaacctaccctttagctgggttcctgccgccaacctgccccccagcctccctgtctccatcctcttctccctgtctccaagggtgctgcttgatccagccactgttcctcctcctgcagtatgccaccacttccttccaccctccagcttccgtccacactgccccagacctggctttcggaaatgctgatggggaaccaaagcccagagaaaggtggtggttcctgcaggttctcagaacccggcacctgcttgccaggcctgggggcggggcacatgcgcactgcagagggttggtgggcaaccggccccatgaatccccaattcatgagcacccccagacacggccatccagccgcttgcccctctcctgggctcaccaagtcaggccccttggccaggtcctcttcacgcaggggttccagccggggggcctgtgagggcacagagtgtgggccgggcctccagcatgggcctggctctggtggataccaggagggtcctcccttgtggggccctggccccacggccctcaccttgcactcgagctggtcgatgagctcctggaggcggttcacctggagccgccactgcatctcggcctctgagctgcgccctgtgtcagaagagccgggggaccaggtggatgaccggctgacactcctcagggctcggcgtcctgcccgccggctgccgcagagcctgctctgcgcctccacgctctctgcatctgaccgccagccatgggcctgggcctccagggtatctgacgccccctccagcgagctctgaagggcttgcagctggctcaccgtctcccgcagcaggaagcgcgtcacaaactggtccactttggaggccctctcgtactccagcttggtggcatccatggcagcgagcactgcacggttcagcgattccaatgcagccagcaccggccggtagacacccaggtgctctgagaagtagtcacacagtttttctgtttctaaattgtcggtgagatgcccatcaatgccgctgaacagttcctgcagctcccccaggctgagaaccccatcggcaaagtaattctggaattcctcaaatgagagcttcccatcatcattcttgtctgctctgcggaaaacgtcctggaagagcgtgtgtccggcgggccccgggtcgggcgcgagctgggggtgccgcggggtctggggctggggctggggcgcgggcggccggagcaggcacacggtgagcagccccgcgcacgccatggcgccgccacccgctcgggctcggctgcggttgctgccgaccctggacgccgcggcggactcggtgtggctagag

SEQ ID NO: 15895 - RNA, 4933 nt, Homo sapiens
  source 1..4933: mol_type = other RNA
gctgggattacaggcatgagccatcacacctggtcgccagattgtttttagtaactgtgcacatatacagcaattacctgcctcaggtgggggctctgatgcatgtttcttgctctgcctgaccttgaatacataattgcttcccgctctgtttgagatttctccttcatgtccaatgaagttgacacttcttactctgcaacagctgtaaaacacccaagtgtcttccacgtcaagattagatgctgccaatgccagagaacacaatacgtactgaagaaactcagctttatctttgaacatctctttctggagccagctcctggcccacaatgtactttagtgagtcttctttacattgttcttatgtaaagactgtttctcacttttcttatcacaacttgtgatgaaacaaagacttcctacatcatagagccgcccgggaggttaaatggactgatgtgtgtaaagcctgtttagaaagttgcctaactcatattaaaccctcaataaatgctagctattatatggttgagctgaaatttttctccgtaaaacatctccatgtatcaaaattggtttctttcttctactaaataattttcttcatttcaaagtattatcatctttatattttcattgttactcaggaatagtttataattttgtatattcattttaagatttatattaagatttaaatctatatccttagtggtgccatctgcactgcaaataattttcagaaaatttttattggcctttttccccaaaaatttcagtcacattgtttggcttttcttcagaataaaacacttcttccagacttaaaaagaagccataactagaaatcctgcaaaaaaatgtcagttttcatgacaaccaaaataagtaaacataaaaacatgtcaaatgttactcagttcctttgaattttctctagttttcatggattattttaagggatagacagtgtttgtttttgtttttgtcttcaggctggaatacatgtttcatgcacctgtatttttacttttttaaaaataatttccttcatctcctcttcagttctcaggcaaaagctttgagttgataatttggggtaaatgacagaatcataggaagatacaatttgatgcacctccagagaatttgacataaataattttagatcaaggagtatctcctattatatccagtaataatattaccttacacttcatagtactttacagttcaaggtacttttccgtacacaatctagtttaaccctaaaaataacccagttacagacatttttaagtgtaatcaaaaatcctcagaaggataaagcaactttcttagagatagcaaatagtgaaacaggaataaaaacccagaatttcttaccctttgtccacttttagtacagtttttcactgttctcagaagaatggctaaaagtttcccttgttacccaccagccattgcagtcatgatactgttccagatgcctagtgtaagtgcatcctgcagaaattgaagatgactaaattcctatcacttgagctgaagtaactttcccaaggtcttatatggaaggtaaattgtcgtagtttctaaatcaatagaaaacaaggcttttcctttcaaaaaatgcattatctagaataagaatcagcaaactctttctgtgaagggcaagatagtgaatattttaggctttgtggactagacagtctctgtgaaactactcaactccattgtagcatgaaagcagccttaagcaatatgtaaatgaatgggcatggctgtgtcccaataaactttatttataaaaacaggagcaggatggatttggctcatgggtggtagtttgcccaccccaatctagaagatgcccacttccattcactctagaaagatggagagtaagatctagattgtccttattgaagcaccaagagaaacacctagcagagggaagtgaattcttatatgttagggttttgttttgttgtcattttatactgggaaggggttgaggaggggctgatctggtaaccctgcaagcctgtattctctaaactgtatgacagaaaatattattcttgcctctggctaggggcctagccagagagatataacagcatacatccttagttctacacatgccacctggtttcttatatattgttctgggagccactgggtacacagagatgaggatggctcattggcaactttctaaaagttaccagcctgcggtagggtagaagaggaggtgatgaggacagacaagtgggcaaaaaaatgcaaagaaaactgtgaaaaccgctactaaggaggtgtttcaaaagtatactgagaagacaaaggtaggagaaatgagctttgtcctgggtgagtagggtggcatgacaggagaggatgacctctagccaggccatgaggaatgtgaggatcccaaaaggagctgatggaagaataagtcaggaagaagaaactgtggcatctgggtacgagatgcaggcatgtgcagaaaatagcataatcccccccacctagagcacgggacaggtgaggagacagagagggagaagcaggagctggaaatccaaccaaaccttcctgagagcctgaaaggtgaagctgggctgttgagattttattccacaacataaaagagcctgggtggttttgagcagatacgtaaggaaaaccagaactgagctttactaagagaatatcaccaggagtgtgggaaaagctaggttcaccaaatgaacctttaagaactccagagcaacactgtccaagagaaatataatgtgaatcccaaatgcaagccatatctgtgaatttaaaatttcttgctagctgcaattttaaacagtaaaaagaaacagaatcagttgtaataatatcgtttagaataatttatccaaaacattatagtttcaatatgtaagcaatataaaaacgataaaggagatattttacattctttacctcgcactaagtcttcgaaatccagagtatattttacatggagagaaaatctcacttcaaatttgcagtatggtaactagcggatgccacataggacaagcacaagtctagagcctaagaaagaagaggcctccaggaagggaccgtaggtgtaagctggaggtgagatcagaggatggttatttgaggatatctggctgcttatttcaccaaatccccttgtgccccaagctcttttagaataaccatcatgggaataattgctgcgcctttaaaaataaactgttcacaaaatactatgcaaacttagaaaatactgttctagctaaaggtaggttaactattaaggtgagtaaaatctcagacactgtatattagggttctctagagggacagaactaataggatagatgtatctataaaaggaggtttattaacgagtattgactcacacaatcataaggtcccacaataggctgtctgcaagctgaggagcaaggaagccagttcaagtcccaaagctgaagaacttggagtctgatatccaagggcaggaggcatccagcacaagagaaagatgtaggctgagaggctaagtgagtctagtcttttcaccttcttctccctgcctttattctggcttccctggcagctgattagaatgtgcccacctagactgatggtgggtctgcctttcccagtccactgactcaaatgttaatctcctttagcaacaccctcacaaacacactcagaaacaatacttttcatctttcaatccaatcaagttgacactcagtattagccatcacagacactttatattacagtggttaaaatatggagtctcaatcttaagatttttcaactggaaaggttcttaactattattttgtaaaaccttccaattttacagatggtggagactcgatatcactcaactagctattactcctgggactccccaattttcttccttttctcttcttttttttttcttcttttttgagacagaatctcactctgtctcccaggctggagtgcaatggtgcaatcttggctcactgcaacctctgcctcctgggttcaagagattctcctgcctcagccttcccaagtatctgggactacaggtgcctgccaccacgcccagccaatttttgtatttttaatagagacggggtttcaccatgttggccaggctagtctcgatctcctgacctcaggtgatccatccgcctcggcctcccaaagtgctgggattacagacatgaggcactgcacccggccccctttttctaggttactctgtgtatgtgtgtgtgtgcatgcgggggttgtgtgtatcacagagagagacagagagagaagacagagacagagccaagcagcagagatgaagtgggggaggaggacagcataacaggatcacggagaggctttttcgagacacaaatgtctgggccccacctgatctactgaatcagagactcacagccagattagatcaataggtagtgccattgctaatctacaaggaggcctatattatcacaggaaatttagcaaaacatagaatagttttaaaccggaattcctgagaggtaaaaagcttattcgaaatattttatcaaactacttggagtgttggcttgtggggcaggaagggagaaggaggagtgagagtgaaaagggactcaaagagacattcatggcacattcagaaataacaatggtcactaaagtccttcatcagagagaggacccaatgatctgcagttttgttgttggtggtggttttttgtttgtgtgtgtgtgtgtgtgtgtgtgtaaaacttggggatgaaactaacctgccatactaagaaaggtaaggttgaggctattatcaactgtcttcatttttcacctccttggcagcagcagcatctcttcaaaaaaa

SEQ ID NO: 15896 - RNA, 1856 nt, Homo sapiens
  source 1..1856: mol_type = other RNA
gctgggattacaggcatgagccatcacatccggctggggaatacttttaaaaacttaaagcgagtgaagggagtctgattaaagtatgcacaataaaatataaagctgtttagaaggcttaaaggtctcggcagtaacctaatttccccactttcctaactttatactagtaattccaaaacatttcctgatgagaaacttcgatttccctgaaattttatgatcactaatagggaaggactgctgagtcacaataatcactggtggaatggggatttaattagcaacaacagtcaagtcccacccagtaagcacctgagagcttgtgagtcagttgaagacacgtatttactgagtacctgccatgtgtaaggtgctggtgatagagcccaaggaacttggttgctatgcttcaaaggagtggtggactgttttactaagtgggatatggcaggaacttgattgaaacacatactcagaagtagttcacctcattatagcttaaatatgtaacactctgggcttcaggtgattccatttcttcctcagttcagatctggtgctgtcagaagcaaagatgtagttgatggattcataagacagatcccacacctgagactgggtcaaattaaatgtttcagctgccagctggtactcttgagaaaggtgtgttgcaaaaacacccttatcatcagtacagatcacagaaggatgggcaatgctgtaccagaatccgaaatggtgctggtcataagatggaactgtctgacttttgacgtttgaggtcaaacagagttccagtggtatccgatgttgcctcacaaagtccaccagatccagggatcctccctcaccggagttgagaaatgttccatgcccgattctgtcaggaagcagatccaggagtatttgtgtttcttttttttggtttggaatagtagggtctccactgaggtcaaggccaagaactgtaccctcagtagaaaggaagaactcctcggcaagttttacagtctccttggctactaaagggccacctcttctgtcaactgctatcaaatacctaacatcaatgtccaagttttcttgtttggactgttttataccttcaagtatagattccacataagtctttttagtcattccagtagcattttctcttctgggtgtgctccttagttccaggtacttgacgccgtcatctgcaaattcttttatgacatcttttgtgaccattagaatatcttcagggctactagtaagctgatgaatagtttgaaacatctggaaacattcttccaaagttcttttctttcccttgtcaatcacagtcatctgatcgtggattttaagatctggcttctgggctattaatttcttcatggtatgagaactaatggatccattcaagtgggcatgaagttccacttttggcaattcagaatagaagtctgtcttgcaaggctgttgctcttctgcctctatcattttagcaggaaaaaaatgattcttctccactcttattcttagtatgagcaatatgatgtatttcagtcagtaaattgtatggtactgaatttccttcagattgctttacttccacacattttggtaagattagctgtatgtgtagatctgggttcagcttcaccagtgagttgtcttctcatttttctgttccttcaacctctccctctccactagctggtttccctcacaggaccaacacgcatgtgcagtatttgcttccacctcttagagatttctcaactacaaggacttaggcaaggtttcccttttgactggaaggcttgtagaaacgtgacaacccgccttccctaacactcatgtcacag

SEQ ID NO: 15897 - RNA, 2064 nt, Homo sapiens
  source 1..2064: mol_type = other RNA
gctgggattacaggcatgagccatcacatccggctggggaatacttttaaaaacttaaagcgagtgaagggagtctgattaaagtatgcacaataaaatataaagctgtttagaaggcttaaaggtctcggcagtaacctaatttccccactttcctaactttatactagtaattccaaaacatttcctgatgagaaacttcgatttccctgaaattttatgatcactaatagggaaggactgctgagtcacaataatcactggtggaatggggatttaattagcaacaacagtcaagtcccacccagtaagcacctgagagcttgtgagtcagttgaagacacgtatttactgagtacctgccatgtgtaaggtgctggtgatagagcccaaggaacttggttgctatgcttcaaaggagtggtggactgttttactaagtgggatatggcaggaacttgattgaaacacatactcagaagtagttcacctcattatagcttaaatatgtaacactctgggcttcaggtgattccatttcttcctcagttcagatctggtgctgtcagaagcaaagatgtagttgatggattcataagacagatcccacacctgagactgggtcaaattaaatgtttcagctgccagctggtactcttgagaaaggtgtgttgcaaaaacacccttatcatcagtacagatcacagaaggatgggcaatgctgtaccagaatccgaaatggtgctggtcataagatggaactgtctgacttttgacgtttgaggtcaaacagagttccagtggtatccgatgttgcctcacaaagtccaccagatccagggatcctccctcaccggagttgagaaatgttccatgcccgattctgtcaggaagcagatccaggagtatttgtgtttcttttttttggtttggaatagtagggtctccactgaggtcaaggccaagaactgtaccctcagtagaaaggaagaactcctcggcaagttttacagtctccttggctactaaagggccacctcttctgtcaactgctatcaaatacctaacatcaatgtccaagttttcttgtttggactgttttataccttcaagtatagattccacataagtctttttagtcattccagtagcattttctcttctgggtgtgctccttagttccaggtacttgacgccgtcatctgcaaattcttttatgacatcttttgtgaccattagaatatcttcagggctactagtaagctgatgaatagtttgaaacatctggaaacattcttccaaagttcttttctttcccttgtcaatcacagtcatctgatcgtggattttaagatctggcttctgggctattaatttcttcatggtatgagaactaatggatccattcaagtgggcatgaagttccacttttggcaattcagaatagaagtctgtcttgcaaggctgttgctcttctgcctctatcattttagcaggaaaaaaatgattcttctccactcttattcttagtatgagcaatatgatgtatttcagtcagtaaattgtatggtactgaatttccttcagattgctttacttccacacattttggtaagattagctgtatgtgtagatctgggttcagcttcacctttttttttttttcttttgagacaggatcttactttgttgcccaggctggagtgcagtgtcacgatcacagcttgctgcagtctcaagcttccagactcaagcgatcctcccacttcagcctccagtgagttgtcttctcatttttctgttccttcaacctctccctctccactagctggtttccctcacaggaccaacacgcatgtgcagtatttgcttccacctcttagagatttctcaactacaaggacttaggcaaggtttcccttttgactggaaggcttgtagaaacgtgacaacccgccttccctaacactcatgtcacagcggtagcggaccgtattctgggacaaatggaactcacgacattccaaagaaaggtcagccgcaagcgaacttagcactggctac

SEQ ID NO: 15898 - RNA, 1937 nt, Homo sapiens
  source 1..1937: mol_type = other RNA
gctgggattacaggcatgagccatcacatccggctggggaatacttttaaaaacttaaagcgagtgaagggagtctgattaaagtatgcacaataaaatataaagctgtttagaaggcttaaaggtctcggcagtaacctaatttccccactttcctaactttatactagtaattccaaaacatttcctgatgagaaacttcgatttccctgaaattttatgatcactaatagggaaggactgctgagtcacaataatcactggtggaatggggatttaattagcaacaacagtcaagtcccacccagtaagcacctgagagcttgtgagtcagttgaagacacgtatttactgagtacctgccatgtgtaaggtgctggtgatagagcccaaggaacttggttgctatgcttcaaaggagtggtggactgttttactaagtgggatatggcaggaacttgattgaaacacatactcagaagtagttcacctcattatagcttaaatatgtaacactctgggcttcaggtgattccatttcttcctcagttcagatctggtgctgtcagaagcaaagatgtagttgatggattcataagacagatcccacacctgagactgggtcaaattaaatgtttcagctgccagctggtactcttgagaaaggtgtgttgcaaaaacacccttatcatcagtacagatcacagaaggatgggcaatgctgtaccagaatccgaaatggtgctggtcataagatggaactgtctgacttttgacgtttgaggtcaaacagagttccagtggtatccgatgttgcctcacaaagtccaccagatccagggatcctccctcaccggagttgagaaatgttccatgcccgattctgtcaggaagcagatccaggagtatttgtgtttcttttttttggtttggaatctctgaaagatgcaatgctaacttcagacctgctttcttagcttctaaaagaggttccaagaagtcttttgcttgtcctacagtagggtctccactgaggtcaaggccaagaactgtaccctcagtagaaaggaagaactcctcggcaagttttacagtctccttggctactaaagggccacctcttctgtcaactgctatcaaatacctaacatcaatgtccaagttttcttgtttggactgttttataccttcaagtatagattccacataagtctttttagtcattccagtagcattttctcttctgggtgtgctccttagttccaggtacttgacgccgtcatctgcaaattcttttatgacatcttttgtgaccattagaatatcttcagggctactagtaagctgatgaatagtttgaaacatctggaaacattcttccaaagttcttttctttcccttgtcaatcacagtcatctgatcgtggattttaagatctggcttctgggctattaatttcttcatggtatgagaactaatggatccattcaagtgggcatgaagttccacttttggcaattcagaatagaagtctgtcttgcaaggctgttgctcttctgcctctatcattttagcaggaaaaaaatgattcttctccactcttattcttagtatgagcaatatgatgtatttcagtcagtaaattgtatggtactgaatttccttcagattgctttacttccacacattttggtaagattagctgtatgtgtagatctgggttcagcttcaccagtgagttgtcttctcatttttctgttccttcaacctctccctctccactagctggtttccctcacaggaccaacacgcatgtgcagtatttgcttccacctcttagagatttctcaactacaaggacttaggcaaggtttcccttttgactggaaggcttgtagaaacgtgacaacccgccttccctaacactcatgtcacag

SEQ ID NO: 15899 - RNA, 2026 nt, Homo sapiens
  source 1..2026: mol_type = other RNA
gctgggattacaggcatgagccatcacatccggctggggaatacttttaaaaacttaaagcgagtgaagggagtctgattaaagtatgcacaataaaatataaagctgtttagaaggcttaaaggtctcggcagtaacctaatttccccactttcctaactttatactagtaattccaaaacatttcctgatgagaaacttcgatttccctgaaattttatgatcactaatagggaaggactgctgagtcacaataatcactggtggaatggggatttaattagcaacaacagtcaagtcccacccagtaagcacctgagagcttgtgagtcagttgaagacacgtatttactgagtacctgccatgtgtaaggtgctggtgatagagcccaaggaacttggttgctatgcttcaaaggagtggtggactgttttactaagtgggatatggcaggaacttgattgaaacacatactcagaagtagttcacctcattatagcttaaatatgtaacactctgggcttcaggtgattccatttcttcctcagttcagatctggtgctgtcagaagcaaagatgtagttgatggattcataagacagatcccacacctgagactgggtcaaattaaatgtttcagctgccagctggtactcttgagaaaggtgtgttgcaaaaacacccttatcatcagtacagatcacagaaggatgggcaatgctgtaccagaatccgaaatggtgctggtcataagatggaactgtctgacttttgacgtttgaggtcaaacagagttccagtggtatccgatgttgcctcacaaagtccaccagatccagggatcctccctcaccggagttgagaaatgttccatgcccgattctgtcaggaagcagatccaggagtatttgtgtttcttttttttggtttggaatctctgaaagatgcaatgctaacttcagacctgctttcttagcttctaaaagaggttccaagaagtcttttgcttgtcctacagtagggtctccactgaggtcaaggccaagaactgtaccctcagtagaaaggaagaactcctcggcaagttttacagtctccttggctactaaagggccacctcttctgtcaactgctatcaaatacctaacatcaatgtccaagttttcttgtttggactgttttataccttcaagtatagattccacataagtctttttagtcattccagtagcattttctcttctgggtgtgctccttagttccaggtacttgacgccgtcatctgcaaattcttttatgacatcttttgtgaccattagaatatcttcagggctactagtaagctgatgaatagtttgaaacatctggaaacattcttccaaagttcttttctttcccttgtcaatcacagtcatctgatcgtggattttaagatctggcttctgggctattaatttcttcatggtatgagaactaatggatccattcaagtgggcatgaagttccacttttggcaattcagaatagaagtctgtcttgcaaggctgttgctcttctgcctctatcattttagcaggaaaaaaatgattcttctccactcttattcttagtatgagcaatatgatgtatttcagtcagtaaattgtatggtactgaatttccttcagattgctttacttccacacattttggtaagattagctgtatgtgtagatctgggttcagcttcacctttttttttttttcttttgagacaggatcttactttgttgcccaggctggagtgcagtgtcacgatcacagcttgctgcagtctcaagcttccagactcaagcgatcctcccacttcagcctccagtgagttgtcttctcatttttctgttccttcaacctctccctctccactagctggtttccctcacaggaccaacacgcatgtgcagtatttgcttccaccgaggtccgtgaggtgtgtgctaaccaaggggcggctcacaaccgtgacagactgccattcctgagtct

SEQ ID NO: 15900 - RNA, 2145 nt, Homo sapiens
  source 1..2145: mol_type = other RNA
gctgggattacaggcatgagccatcacatccggctggggaatacttttaaaaacttaaagcgagtgaagggagtctgattaaagtatgcacaataaaatataaagctgtttagaaggcttaaaggtctcggcagtaacctaatttccccactttcctaactttatactagtaattccaaaacatttcctgatgagaaacttcgatttccctgaaattttatgatcactaatagggaaggactgctgagtcacaataatcactggtggaatggggatttaattagcaacaacagtcaagtcccacccagtaagcacctgagagcttgtgagtcagttgaagacacgtatttactgagtacctgccatgtgtaaggtgctggtgatagagcccaaggaacttggttgctatgcttcaaaggagtggtggactgttttactaagtgggatatggcaggaacttgattgaaacacatactcagaagtagttcacctcattatagcttaaatatgtaacactctgggcttcaggtgattccatttcttcctcagttcagatctggtgctgtcagaagcaaagatgtagttgatggattcataagacagatcccacacctgagactgggtcaaattaaatgtttcagctgccagctggtactcttgagaaaggtgtgttgcaaaaacacccttatcatcagtacagatcacagaaggatgggcaatgctgtaccagaatccgaaatggtgctggtcataagatggaactgtctgacttttgacgtttgaggtcaaacagagttccagtggtatccgatgttgcctcacaaagtccaccagatccagggatcctccctcaccggagttgagaaatgttccatgcccgattctgtcaggaagcagatccaggagtatttgtgtttcttttttttggtttggaatctctgaaagatgcaatgctaacttcagacctgctttcttagcttctaaaagaggttccaagaagtcttttgcttgtcctacagtagggtctccactgaggtcaaggccaagaactgtaccctcagtagaaaggaagaactcctcggcaagttttacagtctccttggctactaaagggccacctcttctgtcaactgctatcaaatacctaacatcaatgtccaagttttcttgtttggactgttttataccttcaagtatagattccacataagtctttttagtcattccagtagcattttctcttctgggtgtgctccttagttccaggtacttgacgccgtcatctgcaaattcttttatgacatcttttgtgaccattagaatatcttcagggctactagtaagctgatgaatagtttgaaacatctggaaacattcttccaaagttcttttctttcccttgtcaatcacagtcatctgatcgtggattttaagatctggcttctgggctattaatttcttcatggtatgagaactaatggatccattcaagtgggcatgaagttccacttttggcaattcagaatagaagtctgtcttgcaaggctgttgctcttctgcctctatcattttagcaggaaaaaaatgattcttctccactcttattcttagtatgagcaatatgatgtatttcagtcagtaaattgtatggtactgaatttccttcagattgctttacttccacacattttggtaagattagctgtatgtgtagatctgggttcagcttcacctttttttttttttcttttgagacaggatcttactttgttgcccaggctggagtgcagtgtcacgatcacagcttgctgcagtctcaagcttccagactcaagcgatcctcccacttcagcctccagtgagttgtcttctcatttttctgttccttcaacctctccctctccactagctggtttccctcacaggaccaacacgcatgtgcagtatttgcttccacctcttagagatttctcaactacaaggacttaggcaaggtttcccttttgactggaaggcttgtagaaacgtgacaacccgccttccctaacactcatgtcacagcggtagcggaccgtattctgggacaaatggaactcacgacattccaaagaaaggtcagccgcaagcgaacttagcactggctac

SEQ ID NO: 15901 - RNA, 2043 nt, Homo sapiens
  source 1..2043: mol_type = other RNA
gctgggattacaggcatgagccatcacatccggctggggaatacttttaaaaacttaaagcgagtgaagggagtctgattaaagtatgcacaataaaatataaagctgtttagaaggcttaaaggtctcggcagtaacctaatttccccactttcctaactttatactagtaattccaaaacatttcctgatgagaaacttcgatttccctgaaattttatgatcactaatagggaaggactgctgagtcacaataatcactggtggaatggggatttaattagcaacaacagtcaagtcccacccagtaagcacctgagagcttgtgagtcagttgaagacacgtatttactgagtacctgccatgtgtaaggtgctggtgatagagcccaaggaacttggttgctatgcttcaaaggagtggtggactgttttactaagtgggatatggcaggaacttgattgaaacacatactcagaagtagttcacctcattatagcttaaatatgtaacactctgggcttcaggtgattccatttcttcctcagttcagatctggtgctgtcagaagcaaagatgtagttgatggattcataagacagatcccacacctgagactgggtcaaattaaatgtttcagctgccagctggtactcttgagaaaggtgtgttgcaaaaacacccttatcatcagtacagatcacagaaggatgggcaatgctgtaccagaatccgaaatggtgctggtcataagatggaactgtctgacttttgacgtttgaggtcaaacagagttccagtggtatccgatgttgcctcacaaagtccaccagatccagggatcctccctcaccggagttgagaaatgttccatgcccgattctgtcaggaagcagatccaggagtatttgtgtttcttttttttggtttggaatctctgaaagatgcaatgctaacttcagacctgctttcttagcttctaaaagaggttccaagaagtcttttgcttgtcctacagtagggtctccactgaggtcaaggccaagaactgtaccctcagtagaaaggaagaactcctcggcaagttttacagtctccttggctactaaagggccacctcttctgtcaactgctatcaaatacctaacatcaatgtccaagttttcttgtttggactgttttataccttcaagtatagattccacataagtctttttagtcattccagtagcattttctcttctgggtgtgctccttagttccaggtacttgacgccgtcatctgcaaattcttttatgacatcttttgtgaccattagaatatcttcagggctactagtaagctgatgaatagtttgaaacatctggaaacattcttccaaagttcttttctttcccttgtcaatcacagtcatctgatcgtggattttaagatctggcttctgggctattaatttcttcatggtatgagaactaatggatccattcaagtgggcatgaagttccacttttggcaattcagaatagaagtctgtcttgcaaggctgttgctcttctgcctctatcattttagcaggaaaaaaatgattcttctccactcttattcttagtatgagcaatatgatgtatttcagtcagtaaattgtatggtactgaatttccttcagattgctttacttccacacattttggtaagattagctgtatgtgtagatctgggttcagcttcacctttttttttttttcttttgagacaggatcttactttgttgcccaggctggagtgcagtgtcacgatcacagcttgctgcagtctcaagcttccagactcaagcgatcctcccacttcagcctccagtgagttgtcttctcatttttctgttccttcaacctctccctctccactagctggtttccctcacaggaccaacacgcatgtgcagtatttgcttccacgacattccaaagaaaggtcagccgcaagcgaacttagcactggctacaccctcctcaattctggttggcgagatgcgctcttcccg

SEQ ID NO: 15902 - RNA, 2040 nt, Homo sapiens
  source 1..2040: mol_type = other RNA
gctgggattacaggcatgagccatcacatccggctggggaatacttttaaaaacttaaagcgagtgaagggagtctgattaaagtatgcacaataaaatataaagctgtttagaaggcttaaaggtctcggcagtaacctaatttccccactttcctaactttatactagtaattccaaaacatttcctgatgagaaacttcgatttccctgaaattttatgatcactaatagggaaggactgctgagtcacaataatcactggtggaatggggatttaattagcaacaacagtcaagtcccacccagtaagcacctgagagcttgtgagtcagttgaagacacgtatttactgagtacctgccatgtgtaaggtgctggtgatagagcccaaggaacttggttgctatgcttcaaaggagtggtggactgttttactaagtgggatatggcaggaacttgattgaaacacatactcagaagtagttcacctcattatagcttaaatatgtaacactctgggcttcaggtgattccatttcttcctcagttcagatctggtgctgtcagaagcaaagatgtagttgatggattcataagacagatcccacacctgagactgggtcaaattaaatgtttcagctgccagctggtactcttgagaaaggtgtgttgcaaaaacacccttatcatcagtacagatcacagaaggatgggcaatgctgtaccagaatccgaaatggtgctggtcataagatggaactgtctgacttttgacgtttgaggtcaaacagagttccagtggtatccgatgttgcctcacaaagtccaccagatccagggatcctccctcaccggagttgagaaatgttccatgcccgattctgtcaggaagcagatccaggagtatttgtgtttcttttttttggtttggaatctctgaaagatgcaatgctaacttcagacctgctttcttagcttctaaaagaggttccaagaagtcttttgcttgtcctacagtagggtctccactgaggtcaaggccaagaactgtaccctcagtagaaaggaagaactcctcggcaagttttacagtctccttggctactaaagggccacctcttctgtcaactgctatcaaatacctaacatcaatgtccaagttttcttgtttggactgttttataccttcaagtatagattccacataagtctttttagtcattccagtagcattttctcttctgggtgtgctccttagttccaggtacttgacgccgtcatctgcaaattcttttatgacatcttttgtgaccattagaatatcttcagggctactagtaagctgatgaatagtttgaaacatctggaaacattcttccaaagttcttttctttcccttgtcaatcacagtcatctgatcgtggattttaagatctggcttctgggctattaatttcttcatggtatgagaactaatggatccattcaagtgggcatgaagttccacttttggcaattcagaatagaagtctgtcttgcaaggctgttgctcttctgcctctatcattttagcaggaaaaaaatgattcttctccactcttattcttagtatgagcaatatgatgtatttcagtcagtaaattgtatggtactgaatttccttcagattgctttacttccacacattttggtaagattagctgtatgtgtagatctgggttcagcttcacctttttttttttttcttttgagacaggatcttactttgttgcccaggctggagtgcagtgtcacgatcacagcttgctgcagtctcaagcttccagactcaagcgatcctcccacttcagcctcctcttagagatttctcaactacaaggacttaggcaaggtttcccttttgactggaaggcttgtagaaacgtgacaacccgccttccctaacactcatgtcacagcggtagcggaccgtattctgggacaaatggaactcacgacattccaaagaaaggtcagccgcaagcgaacttagcactgg

SEQ ID NO: 15903 - RNA, 1711 nt, Homo sapiens
  source 1..1711: mol_type = other RNA
gctgggattacaggcatgagccatcacatccggctggggaatacttttaaaaacttaaagcgagtgaagggagtctgattaaagtatgcacaataaaatataaagctgtttagaaggcttaaaggtctcggcagtaacctaatttccccactttcctaactttatactagtaattccaaaacatttcctgatgagaaacttcgatttccctgaaattttatgatcactaatagggaaggactgctgagtcacaataatcactggtggaatggggatttaattagcaacaacagtcaagtcccacccagtaagcacctgagagcttgtgagtcagttgaagacacgtatttactgagtacctgccatgtgtaaggtgctggtgatagagcccaaggaacttggttgctatgcttcaaaggagtggtggactgttttactaagtgggatatggcaggaacttgattgaaacacatactcagaagtagttcacctcattatagcttaaatatgtaacactctgggcttcaggtgattccatttcttcctcagttcagatctggtgctgtcagaagcaaagatgtagttgatggattcataagacagatcccacacctgagactgggtcaaattaaatgtttcagctgccagctggtactcttgagaaaggtgtgttgcaaaaacacccttatcatcagtacagatcacagaaggatgggcaatgctgtaccagaatccgaaatggtgctggtcataagatggaactgtctgacttttgacgtttgaggtcaaacagagttccagtggtatccgatgttgcctcacaaagtccaccagatccagggatcctccctcaccggagttgagaaatgttccatgcccgattctgtcaggaagcagatccaggagtatttgtgtttcttttttttggtttggaatctctgaaagatgcaatgctaacttcagacctgctttcttagcttctaaaagaggttccaagaagtcttttgcttgtcctacagtagggtctccactgaggtcaaggccaagaactgtaccctcagtagaaaggaagaactcctcggcaagttttacagtctccttggctactaaagggccacctcttctgtcaactgctatcaaatacctaacatcaatgtccaagttttcttgtttggactgttttataccttcaagtatagattccacataagtctttttagtcattccagtagcattttctcttctgggtgtgctccttagttccaggtacttgacgccgtcatctgcaaattcttttatgacatcttttgtgaccattagaatatcttcagggctactagtaagctgatgaatagtttgaaacatctggaaacattcttccaaagttcttttctttcccttgtcaatcacagtcatctgatcgtggattttaagatctggcttctgggctattaatttcttcatggtatgagaactaatggatccattcaagtgggcatgaagttccagtgagttgtcttctcatttttctgttccttcaacctctccctctccactagctggtttccctcacaggaccaacacgcatgtgcagtatttgcttccacctcttagagatttctcaactacaaggacttaggcaaggtttcccttttgactggaaggcttgtagaaacgtgacaacccgccttccctaacactcatgtcacag

SEQ ID NO: 15904 - RNA, 1755 nt, Homo sapiens
  source 1..1755: mol_type = other RNA
gctgggattacaggcatgagccatcacatccggctggggaatacttttaaaaacttaaagcgagtgaagggagtctgattaaagtatgcacaataaaatataaagctgtttagaaggcttaaaggtctcggcagtaacctaatttccccactttcctaactttatactagtaattccaaaacatttcctgatgagaaacttcgatttccctgaaattttatgatcactaatagggaaggactgctgagtcacaataatcactggtggaatggggatttaattagcaacaacagtcaagtcccacccagtaagcacctgagagcttgtgagtcagttgaagacacgtatttactgagtacctgccatgtgtaaggtgctggtgatagagcccaaggaacttggttgctatgcttcaaaggagtggtggactgttttactaagtgggatatggcaggaacttgattgaaacacatactcagaagtagttcacctcattatagcttaaatatgtaacactctgggcttcaggtgattccatttcttcctcagttcagatctggtgctgtcagaagcaaagatgtagttgatggattcataagacagatcccacacctgagactgggtcaaattaaatgtttcagctgccagctggtactcttgagaaaggtgtgttgcaaaaacacccttatcatcagtccagtggtatccgatgttgcctcacaaagtccaccagatccagggatcctccctcaccggagttgagaaatgttccatgcccgattctgtcaggaagcagatccaggagtatttgtgtttcttttttttggtttggaatagtagggtctccactgaggtcaaggccaagaactgtaccctcagtagaaaggaagaactcctcggcaagttttacagtctccttggctactaaagggccacctcttctgtcaactgctatcaaatacctaacatcaatgtccaagttttcttgtttggactgttttataccttcaagtatagattccacataagtctttttagtcattccagtagcattttctcttctgggtgtgctccttagttccaggtacttgacgccgtcatctgcaaattcttttatgacatcttttgtgaccattagaatatcttcagggctactagtaagctgatgaatagtttgaaacatctggaaacattcttccaaagttcttttctttcccttgtcaatcacagtcatctgatcgtggattttaagatctggcttctgggctattaatttcttcatggtatgagaactaatggatccattcaagtgggcatgaagttccacttttggcaattcagaatagaagtctgtcttgcaaggctgttgctcttctgcctctatcattttagcaggaaaaaaatgattcttctccactcttattcttagtatgagcaatatgatgtatttcagtcagtaaattgtatggtactgaatttccttcagattgctttacttccacacattttggtaagattagctgtatgtgtagatctgggttcagcttcaccagtgagttgtcttctcatttttctgttccttcaacctctccctctccactagctggtttccctcacaggaccaacacgcatgtgcagtatttgcttccacctcttagagatttctcaactacaaggacttaggcaaggtttcccttttgactggaaggcttgtagaaacgtgacaacccgccttccctaacactcatgtcacag

SEQ ID NO: 15905 - RNA, 4032 nt, Homo sapiens
  source 1..4032: mol_type = other RNA
gctgggattacaggcatgagccatcacgcccggccaaagttttagaatttaagttattccaaaaaaaattttttttttcaaaaatacagactgcatccaattaaattctatgttaactggtaatgactaggtctaaaatgttaggtatttaccaataaatgacataaaataactcaacaacaaagggatttttttttttaagagatagggtctcactttatcactcaggtttggctgagggcagtggtgtgatcacagctcactgaagcctccaactcctgggctcaagtgatcctcccgcctcagtctaccagagtatattcttgaaagtaaaattacaaatgaaattcagcagtgttaaaaataagcccacttgcagacaattatcatttttcttcctttctttcctcactatctgtacttggcatatttcctacagtggctgtcttaaagaaaaaaaggaatccttcacaaatagtgtagccaaaaaagttggactaatatacaatgctatcagtaaagtattatatataaaatttataagtgctaaagtgtaattttgaaagacacttaagatactccttttttttttgagacaaggtctcagccctgtcgcccaggctggagtgcactagcacaacatcagctcactgcaacctccgcctcccaggttcaagcgattctcctgcctcagcctcccaagtagctgagactacaggcgcacgccagcatgtccagataattttttgtatttttagtagagatggggtttcaccatgttggccaggatggtctcaaatctcttgacctcgtgatctgcccatgtcggcttcccaaagtgttaggataacaggcatgagctaccgtgcccagcctacttaaaatattcttgaaatagctctccccacctccttttttttttttttttgagaatgagtttcactcgacacccaggctggagtgcagtggtgcgatcttggctcactgcaacctctgcctcccaggttcaagcgattatcctgcctcagcctcctgagtagctgggattacaaatgtgcaccaccacatctggctaattttttttttttttttttgtatttttagtagagacggggtttcaccaagttggcctggctggtctcgaacacctgacctcaattgatccacctgcctcggcctcccaaagtattataggcatgagccaccgagcccggccttttttgttttttgtttttttaaaggcagggttttgctctgttgcccaggctggagtgcagtggtgtgatcacagatcactgcagccttgacctctcctggtctcaagtgatcctcccacctcagccttcagaacagctgggactacaggtgtgtgtcaccatgcccagtaatttttttgtatatttgtagaggcagggtctcccaatgttgcctgggctggtctcaaactcctgggctcaagcaatccaccagctttggccttccaaagttctaggattatacgcatgagccactgtgccctgccccaatattttgttacttactagtgagactaaacacttttctaaaagtttgttagccatactatcctataaaagctgtttgttcatgtcttttgtccatttatctttttttttgtttttcttgagacagagtcttgctctgtggcccaggctggagtgcaggggtgcaatctcggctcactgcaagctccgcctcccaggttcaaatgattctcctgcctcagcctcctgagtagctgggattacaggcatgtgccaccatgcccagctaatttttttgtgtgtgtttttcagtagagatggggtttcaccatgttggccaggctgatctcgaattcctgacctcaggtgctccacccgcctcagcctcccaaagtactgggattacaggggtgagccaccgcacccggccaattttctgtatttttaatagagacagggtttcatcctgttggccaggctggcctcgaacttcggacctcaggtgatccacccgcctcgacctcccaaagtgctgggattacaggtgtgggccaccacacccagccaatttttttgtatttttagtagagacagggtttcatcatgttggccaggctggtcgcaaactcctgacctcaggtgatccacccgcctcagcatcccaaagtgctgggattacaggcatgagccaccactcccggccaatgttttgtatttttagtagagatggggtttcatcatgttggccagactggtctcaaactctggacctcaggtgatccacctgcctcagcctcccaaagtgtagggattacaggtgtgagccaccgcgcccagcctatgtttctattttatacatattcaacaaacatgattccccaacttctgcaaaataatttctttttcaagaacattgattttagagctcacactaagaaaaagaatacaaaaataatggcatagaaagtgaaaaaacaaaaataaaaagtagaaagctaaagtttcccattaaaatgatcaatatactgtgcagtaagtcaaatgtgtacaatgaattaagaaaatatgatatataaaaatccaaatttacaaaattaagtacaaataggtgtttatattacaaagtgatactggtttataaaaggattcaacatagattttttttaaatggttgttttcctcaatcaatttaacaatgattttaaatgtataaaattttaatatctctttgagacagtgatccaagcttcttcccttgatgatgttaccagttcatactttgtttcaataacctgtccctccacagaaagtaggtgcagtctcttcaccaatacactaagaagtactgtggtcaccatatatgcaaacctcaactctggacactcctgtgtgcctgagaatccaagtgaggaaaaagttttcattactaattcatcatcaaaccgatctggatcaaacttgtgtggagatggccaagtattaggatcctgaagtaccacaccaagggcataaaggacgagggtctctctaggaataataaatcggtcaatttttccttcaatatcttgaagctgggcagaaactggagtcagtttggcagttcgaacagtttcacaaagcacatgctgacaatatattttgcagttattatgcaactggccagagaaaatatcatactgtcttctaggatctgttggtcattaaggttcccttgtactaaggagtcaatgaaaatatgttgactgaagttccttccttttcgttcttttatgatgttccttaaaacagactccagttgcatgagggcatcttcatattgttttttccgagtcatgtttttatcaagtgacccatctagaaagccttttccaatctcagaccaaactgtgccatgattcttctggaagcgaatgacttcctgatcatcttcaaatgtactacccattaccatctgtgtaacagacttcatagcaaaaccaagcatatgctggctgaggggcacgtgctgggtctctgggtaggagagccatttatctaataattcttctgaaagctttaggaggagggcaaagttactcttcagagaatcagtcacaccattttcatacaattttttcctcatgtggttttcactcacactgccaccaccagattgataccttaataatgacttcagcatggtttcaaaagggtccgatgtcttattgggattgatatgctgcttcagtacatcaacagtgcccaaactaaccacgaggcgcctgccaaaccagaaggagaccacaggcccatatctctcatgcaaattaaccaggaactcatgcaaacttccactattcacaatatctggaagattaccatctttttcttcagttggagtaatccctggaattcctgcagcttgtctggaagccggatagaggtagagcacggctcccaccaacgccagcaagaaggtaacggcgaagatcgcgaagtccaacatggttctgccgcccagggagccacgtctcggatcggccgctccagc

SEQ ID NO: 15906 - RNA, 3953 nt, Homo sapiens
  source 1..3953: mol_type = other RNA
gctgggattacaggcatgagccatcacgcccggccaaagttttagaatttaagttattccaaaaaaaattttttttttcaaaaatacagactgcatccaattaaattctatgttaactggtaatgactaggtctaaaatgttaggtatttaccaataaatgacataaaataactcaacaacaaagggatttttttttttaagagatagggtctcactttatcactcaggtttggctgagggcagtggtgtgatcacagctcactgaagcctccaactcctgggctcaagtgatcctcccgcctcagtctaccagagtatattcttgaaagtaaaattacaaatgaaattcagcagtgttaaaaataagcccacttgcagacaattatcatttttcttcctttctttcctcactatctgtacttggcatatttcctacagtggctgtcttaaagaaaaaaaggaatccttcacaaatagtgtagccaaaaaagttggactaatatacaatgctatcagtaaagtattatatataaaatttataagtgctaaagtgtaattttgaaagacacttaagatactccttttttttttgagacaaggtctcagccctgtcgcccaggctggagtgcactagcacaacatcagctcactgcaacctccgcctcccaggttcaagcgattctcctgcctcagcctcccaagtagctgagactacaggcgcacgccagcatgtccagataattttttgtatttttagtagagatggggtttcaccatgttggccaggatggtctcaaatctcttgacctcgtgatctgcccatgtcggcttcccaaagtgttaggataacaggcatgagctaccgtgcccagcctacttaaaatattcttgaaatagctctccccacctccttttttttttttttttgagaatgagtttcactcgacacccaggctggagtgcagtggtgcgatcttggctcactgcaacctctgcctcccaggttcaagcgattatcctgcctcagcctcctgagtagctgggattacaaatgtgcaccaccacatctggctaattttttttttttttttttgtatttttagtagagacggggtttcaccaagttggcctggctggtctcgaacacctgacctcaattgatccacctgcctcggcctcccaaagtattataggcatgagccaccgagcccggccttttttgttttttgtttttttaaaggcagggttttgctctgttgcccaggctggagtgcagtggtgtgatcacagatcactgcagccttgacctctcctggtctcaagtgatcctcccacctcagccttcagaacagctgggactacaggtgtgtgtcaccatgcccagtaatttttttgtatatttgtagaggcagggtctcccaatgttgcctgggctggtctcaaactcctgggctcaagcaatccaccagctttggccttccaaagttctaggattatacgcatgagccactgtgccctgccccaatattttgttacttactagtgagactaaacacttttctaaaagtttgttagccatactatcctataaaagctgtttgttcatgtcttttgtccatttatctttttttttgtttttcttgagacagagtcttgctctgtggcccaggctggagtgcaggggtgcaatctcggctcactgcaagctccgcctcccaggttcaaatgattctcctgcctcagcctcctgagtagctgggattacaggcatgtgccaccatgcccagctaatttttttgtgtgtgtttttcagtagagatggggtttcaccatgttggccaggctgatctcgaattcctgacctcaggtgctccacccgcctcagcctcccaaagtactgggattacaggggtgagccaccgcacccggccaattttctgtatttttaatagagacagggtttcatcctgttggccaggctggcctcgaacttcggacctcaggtgatccacccgcctcgacctcccaaagtgctgggattacaggtgtgggccaccacacccagccaatttttttgtatttttagtagagacagggtttcatcatgttggccaggctggtcgcaaactcctgacctcaggtgatccacccgcctcagcatcccaaagtgctgggattacaggcatgagccaccactcccggccaatgttttgtatttttagtagagatggggtttcatcatgttggccagactggtctcaaactctggacctcaggtgatccacctgcctcagcctcccaaagtgtagggattacaggtgtgagccaccgcgcccagcctatgtttctattttatacatattcaacaaacatgattccccaacttctgcaaaataatttctttttcaagaacattgattttagagctcacactaagaaaaagaatacaaaaataatggcatagaaagtgaaaaaacaaaaataaaaagtagaaagctaaagtttcccattaaaatgatcaatatactgtgcagtaagtcaaatgtgtacaatgaattaagaaaatatgatatataaaaatccaaatttacaaaattaagtacaaataggtgtttatattacaaagtgatactggtttataaaaggattcaacatagattttttttaaatggttgttttcctcaatcaatttaacaatgattttaaatgtataaaattttaatatctctttgagacagtgatccaagcttcttcccttgatgatgttaccagttcatactttgtttcaataacctgtccctccacagaaagtaggtgcagtctcttcaccaatacactaagaagtactgtggtcaccatatatgcaaacctcaactctggacactcctgtgtgcctgagaatccaagtgaggaaaaagttttcattactaattcatcatcaaaccgatctggatcaaacttgtgtggagatggccaagtattaggatcctgaagtaccacaccaagggcataaaggacgagggtctctctaggaataataaatcggtcaatttttccttcaatatcttgaagctgggcagaaactggagtcagtttggcagttcgaacagtttcacaaagcacatgctgacaatatattttgcagttattatgcaactggccagagaaaatatcatactgtcttctaggatctgttggtcattaaggttcccttgtactaaggagtcaatgaaaatatgttgactgaagttccttccttttcgttcttttatgatgttccttaaaacagactccagttgcatgagggtgtgccatgattcttctggaagcgaatgacttcctgatcatcttcaaatgtactacccattaccatctgtgtaacagacttcatagcaaaaccaagcatatgctggctgaggggcacgtgctgggtctctgggtaggagagccatttatctaataattcttctgaaagctttaggaggagggcaaagttactcttcagagaatcagtcacaccattttcatacaattttttcctcatgtggttttcactcacactgccaccaccagattgataccttaataatgacttcagcatggtttcaaaagggtccgatgtcttattgggattgatatgctgcttcagtacatcaacagtgcccaaactaaccacgaggcgcctgccaaaccagaaggagaccacaggcccatatctctcatgcaaattaaccaggaactcatgcaaacttccactattcacaatatctggaagattaccatctttttcttcagttggagtaatccctggaattcctgcagcttgtctggaagccggatagaggtagagcacggctcccaccaacgccagcaagaaggtaacggcgaagatcgcgaagtccaacatggttctgccgcccagggagccacgtctcggatcggccgctccagc

SEQ ID NO: 15907 - RNA, 3736 nt, Homo sapiens
  source 1..3736: mol_type = other RNA
gctgggattacaggcatgagccatcacgcccggccaaagttttagaatttaagttattccaaaaaaaattttttttttcaaaaatacagactgcatccaattaaattctatgttaactggtaatgactaggtctaaaatgttaggtatttaccaataaatgacataaaataactcaacaacaaagggatttttttttttaagagatagggtctcactttatcactcaggtttggctgagggcagtggtgtgatcacagctcactgaagcctccaactcctgggctcaagtgatcctcccgcctcagtctaccagagtatattcttgaaagtaaaattacaaatgaaattcagcagtgttaaaaataagcccacttgcagacaattatcatttttcttcctttctttcctcactatctgtacttggcatatttcctacagtggctgtcttaaagaaaaaaaggaatccttcacaaatagtgtagccaaaaaagttggactaatatacaatgctatcagtaaagtattatatataaaatttataagtgctaaagtgtaattttgaaagacacttaagatactccttttttttttgagacaaggtctcagccctgtcgcccaggctggagtgcactagcacaacatcagctcactgcaacctccgcctcccaggttcaagcgattctcctgcctcagcctcccaagtagctgagactacaggcgcacgccagcatgtccagataattttttgtatttttagtagagatggggtttcaccatgttggccaggatggtctcaaatctcttgacctcgtgatctgcccatgtcggcttcccaaagtgttaggataacaggcatgagctaccgtgcccagcctacttaaaatattcttgaaatagctctccccacctccttttttttttttttttgagaatgagtttcactcgacacccaggctggagtgcagtggtgcgatcttggctcactgcaacctctgcctcccaggttcaagcgattatcctgcctcagcctcctgagtagctgggattacaaatgtgcaccaccacatctggctaattttttttttttttttttgtatttttagtagagacggggtttcaccaagttggcctggctggtctcgaacacctgacctcaattgatccacctgcctcggcctcccaaagtattataggcatgagccaccgagcccggccttttttgttttttgtttttttaaaggcagggttttgctctgttgcccaggctggagtgcagtggtgtgatcacagatcactgcagccttgacctctcctggtctcaagtgatcctcccacctcagccttcagaacagctgggactacaggtgtgtgtcaccatgcccagtaatttttttgtatatttgtagaggcagggtctcccaatgttgcctgggctggtctcaaactcctgggctcaagcaatccaccagctttggccttccaaagttctaggattatacgcatgagccactgtgccctgccccaatattttgttacttactagtgagactaaacacttttctaaaagtttgttagccatactatcctataaaagctgtttgttcatgtcttttgtccatttatctttttttttgtttttcttgagacagagtcttgctctgtggcccaggctggagtgcaggggtgcaatctcggctcactgcaagctccgcctcccaggttcaaatgattctcctgcctcagcctcctgagtagctgggattacaggcatgtgccaccatgcccagctaatttttttgtgtgtgtttttcagtagagatggggtttcaccatgttggccaggctgatctcgaattcctgacctcaggtgctccacccgcctcagcctcccaaagtactgggattacaggggtgagccaccgcacccggccaattttctgtatttttaatagagacagggtttcatcctgttggccaggctggcctcgaacttcggacctcaggtgatccacccgcctcgacctcccaaagtgctgggattacaggtgtgggccaccacacccagccaatttttttgtatttttagtagagacagggtttcatcatgttggccaggctggtcgcaaactcctgacctcaggtgatccacccgcctcagcatcccaaagtgctgggattacaggcatgagccaccactcccggccaatgttttgtatttttagtagagatggggtttcatcatgttggccagactggtctcaaactctggacctcaggtgatccacctgcctcagcctcccaaagtgtagggattacaggtgtgagccaccgcgcccagcctatgtttctattttatacatattcaacaaacatgattccccaacttctgcaaaataatttctttttcaagaacattgattttagagctcacactaagaaaaagaatacaaaaataatggcatagaaagtgaaaaaacaaaaataaaaagtagaaagctaaagtttcccattaaaatgatcaatatactgtgcagtaagtcaaatgtgtacaatgaattaagaaaatatgatatataaaaatccaaatttacaaaattaagtacaaataggtgtttatattacaaagtgatactggtttataaaaggattcaacatagattttttttaaatggttgttttcctcaatcaatttaacaatgattttaaatgtataaaattttaatatctctttgagacagtgatccaagcttcttcccttgatgatgttaccagttcatactttgtttcaataacctgtccctccacagaaagtaggtgcagtctcttcaccaatacactaagaagtactgtggtcaccatatatgcaaacctcaactctggacactcctgtgtgcctgagaatccaagtgaggaaaaagttttcattactaattcatcatcaaaccgatctggatcaaacttgtgtggagatggccaagtattaggatcctgaagtaccacaccaagggcataaaggacgagggtctctctaggaataataaatcggtcaatttttccttcaatatcttgaagctgggcagaaactggagtcagtttggcagttcgaacagtttcacaaagcacatgctgacaatatattttgcagttattatgcaactggccagagaaaatatcatactgtcttctaggatctgttggtcattaaggttcccttgtactaaggagtcaatgaaaatatgttgactgaagttccttccttttcgttcttttatgatgttccttaaaacagactccagttgcatgagggtgtgccatgattcttctggaagcgaatgacttcctgatcatcttcaaatgtactacccattaccatctgtgtaacagacttcatagcaaaaccaagcatatgctggctgaggggcacgtgctgggtctctgggtaggagagccatttatctaataattcttctgaaagctttaggaggagggcaaagttactcttcagagaatcagtcacaccattttcatacaattttttcctcatgtggttttcactcacactgccaccaccagattgataccttaataatgacttcagcatggtttcaaaagggtccgcggatagaggtagagcacggctcccaccaacgccagcaagaaggtaacggcgaagatcgcgaagtccaacatggttctgccgcccagggagccacgtctcggatcggccgctccagc
